European Patent Application EP 4 458 963 A1, published November 6, 2024. Title: Highly active CRISPR base editors obtained through Cas-assisted substrate-linked directed evolution (CaSLiDE). Applicant: Technische Universität Dresden. The sequence listing filed with the application follows.

SEQUENCE LISTING (3550 sequences)

SEQ ID NO: 1 - protein, 726 aa, Homo sapiens
SEVEFSHEYWMRHALTLAKRARDEREVPVGAVLVLNNRVIGEGWNRAIGLHDPTAHAEIMALRQGGLVMQNYRLIDATLYVTFEPCVMCAGAMIHSRIGRVVFGVRNSKRGAAGSLMNVLNYPGMNHRVEITEGILADECAALLCDFYRMPRQVFNAQKKAQSSINSGGSSGGSSGSETPGTSESATPESSGGSSGGSAKNTITKTLKLRIVRPYNSAEVEKIVADEKNNREKIALEKNKDKVKEACSKHLKVAAYCTTQVERNACLFCKARKLDDKFYQKLRGQFPDAVFWQEISEIFRQLQKQAAEIYNQSLIELYYEIFIKGKGIANASSVEHYLSDVCYTRAAELFKNAAIASGLRSKIKSNFRLKELKNMKSGLPTTKSDNFPIPLVKQKGGQYTGFEISNHNSDFIIKIPFGRWQVKKEIDKYRPWEKFDFEQVQKSPKPISLLLSTQRRKRNKGWSKDEGTEAEIKKVMNGDYQTSYIEVKRGSKIGEKSAWMLNLSIDVPKIDKGVDPSIIGGIDVGVKSPLVCAINNAFSRYSISDNDLFHFNKKMFARRRILLKKNRHKRAGHGAKNKLKPITILTEKSERFRKKLIERWACEIADFFIKNKVGTVQMENLESMKRKEDSYFNIRLRGFWPYAEMQNKIEFKLKQYGIEIRKVAPNNTSKTCSKCGHLNNYFNFEYRKKNKFPHFKCEKCNFKENADYNAALNISNPKLKSTKEEP

SEQ ID NO: 2 - protein, 726 aa, synthetic construct
SEVEFSHEYWMRHALTLAKRARDEREVPVGAILVLNNRVIGEGWNRAIGLHDPTAHAEIMALRQGGLVMQNYRLIDATLYVTFEPCVMCAGAMIHSRIGRVVFGVRNSKHGAAGSLMNVLNYPGMNHRVEITEGILADECAALLCDFYRMPRQVFNARKKTQSSINPGGPSGGSSGSETPDTSESATPESSGGNTGGSAKNTITKTLKLRIVRPYNSAEVEKIVADEKNNREKIALEKNKDKVKEACSEHLKVAAYCTTQVERNACLFCKARKLDDKFYQKLRGQFPDAVFWQELGGIFRQLQKQAAEIYNQSLIELYYEIFIKGKGITNTSRVEHYLSDVCYTRAAELFKNAAIASGLRGKVKSNFRLKELKNMKSGLPTTKSDNFPIPLVKQKGGQYTGFEISSHNDDFIIKIPFGRWQVKEEIDKYRPWEKFDFEQVRKNPKPISLLLSTQRRKRNKGWSKDEGTEAEIRKVMNGDYQTSYIEVKRGSKIGEKSAWMLNLSIDVPKIDKGVDPSIIGGIDVGVRSPLVCAINNAFSRYSISDNELFHFNKKMFARRRILLKKNRHKRAGHGAKNKLKPIAIMTEKSKRFRKKLIERWACEIADFFIKNKVGTVQMENLESMKRKEDSYFNIRLRGFWPYAEMQNKIEFKLKQYGIVVRKVAPNNTSKTCSKCGHLNNYFNFEYRKKNKFPHFKCEKCNFKENADYNAALNISNPKLKSTKGEP

SEQ ID NO: 3 - protein, 726 aa, synthetic construct
SEVEFSHEYWMRHALALAKRARDEREVPVGAVLVLNNRVIGEGWNRTAGLHDPTAHAEIMALRQGGLVMQNHRLVDATLYVTFEPCVLCAGAMVHSRIGRVVFGVRNSKRGAAGSLMNVLNYPGMNHRVEITEGILADECAALLCDFYRMPRQVFNAQKKAQSNINSGGSPGGSSGCETPGTSESPTPESSGGCSGGSAKNTITKTLQLRIVRPYNSAEVEKVVADEKNNREKIALEKNKDKVKEACSKHLKMASYCTTQVERNACLFCKARKLDDKFYQKLRGQFPDAVFWQELGGIFRQLQKQAAEIYNQSLIELYYEIFIKGKGITNASRVEHYLSDVCYTRAAELFKNAAIASGLRNKIKSNFRLKELRNMKSGLPTTKSDNFPIPLVKQKGGQYTGFEIGNHNGDFIIKIPFGRWQAKKEIDKYRPWEKFDFEQVRKSPKPISLLLSTQRRKRNKGWSKDEGTEAEIRKVMNGDYQTSYIEVKRGSKTGEKSAWMLNLSIDVPKIDKGVDPSIIGGIDVGVKSPLVCAINNAFSRYGISDNDLFRFNKKMFARRRILLKKNRHKRAGHGARNKLKPITVLTEKSERFRKKLIERWACEIANFFIKNKVGTVQMENLESMKRREDSYFNIRLRGFWPYAEMQSKIEFKLKQYGIKIRKVAPNNTSKTCSKCGHLNNYFNFEFRKKNKFPHFKCEKCNFKEDADYNAALNISNPKLKSTKEEP

SEQ ID NO: 4 - protein, 726 aa, synthetic construct
SEVEFSHEYWMRHALTLAKRARDEREVPVGAVLVLNNRVIGEGWNRAIGLHDPTAHAEIMALRQGGLVMQNYRLTDATLYVTFEPCVMCAGAMIHSRIGRVVFGVRNSKRGAAGSLMNVLNYPGMNHCVEITEGILVDECAALLCDFYRMPRQVLNAQKKAQSSISSGGSSGGSSGSETPGASGSVTPKSSGGSSAGSTKDTITKTLKLRIVRPYNSAEVEKIVADEKNSREKIALEKNKDKVKEACSKHLKVASYCTTQVERNACLFCKARKLDDKFYQKLRGQFPDAVFWQELGEIFRQLQKQAAEIYNQSLIELYYEIFIKGKGFANASSVEHYLSDVCYTRAAELFKNAAIASGLRGKVKSNFRLKELKNMKSGLPTTKSDNFPIPLVKQKGGQYTGFEISSHNDDFIIKIPFGRWQVKKEIDKYRPWEKFDFEQVRKSPKPISLLLSTQRRKRNKGWSKDEGTEAEIRRVMNGDYQTSYIEVKRGSKIGEKSAWMLNLSIDVPKIDKGVDPSIIGGVDVGVKSPLVCAINNAFSRYSISDNDLFHFNKKMFARRRILLRKNRHKRAGHGAKNKLKPITIMTEKSKRFRKKLIERWACEIADFFIKNKVGTVQMENLESMKRKEDSYFNIRLRGFWPYAEMQNKIEFKLKQYGIVVRKVAPNNTSKTCSKCGHLNNHFNFEYRKKNKFPHFKCEKCNFKENADYNAALNISNPKLKSTKEEP

SEQ ID NO: 5 - protein, 726 aa, synthetic construct
SEVVFSHEYWMRHALTLAKRARDEREVPVGAILVLNDRVIGEGWNRAIGLHDPTAHAEIMALRQGGLVMQNYRLIDATLYVTFEPCVMCAGAMIHSRIGRVVFGVRNSKHGAAGSLMNVLNYPGMNHRVEITEGILADECAALLCDFYRMPRQVFNARKKARSNINSGGSSGGSSGSETLGTREGATPKSSGGSSAGSTKNTITKTLKLRIVRPYNSAEVEKIVADEKNSREKIALEKNKDKVKEACSEHLKVAAYCTTQVERNACLFCKARKLDDRFYQKLRGQFPDAVFWQETGEIFRQLQRQAAEIYNQSLIELYYEIFIKGKGFANASSVEHYLSDVCYTRAAELFKNAAIASGLRGKVKSNFRLKELKNMKSGLPTTKSDNFPIPLVKQKGGQYTGFEISSHNDDFIIKIPFGRWQMKKEIDRYRPWEKFDFEQVRKSPKPISLLLSTQRRKRNKGWSRDEGTEAEIRKVMNGDYQTSYIEVKRGSKIGEKSAWMLSLSIDVPKIDKGVDPSIIGGIDVGVKSPLVCAINNAFCRYSISDNDLFHFNKKMFARRRILLKKSRHKRAGHGAKNKLKPISILTEKSKRFRKKLIERWACEIADFFIKNKVGTVQMENLESMKRKEDSYFNIRLRGFWPYAEMQNKIEFKLKQYGIEVRKVAPNNTSKTCSKCGHLNNYFNFEYRKKNKFPHFKCEKCNFKENADYNAALNISNPKLKSTREEP

SEQ ID NO: 6 - protein, 726 aa, synthetic construct
SEVEFSHEYWMRRALTLAKRARDEREVPVGAVLVLNNRVIGVGWNRAVGLHDPTAHAEIMALRQGGLVMQNYRLIEATLYVTFEPCIMCAGAMIHSRIGRVVFGVRNSKRGAAGSLMNVLNYPGMNHRVEVTEGILADECAALLCDYYRMPRQVFNARKKAQSSINSGGSSDGGSGNETPGTSESATPESSGGNSGGSAKNTITKTLKLRIVRPYNSAEVEKIVADEKNNREKVALEKNKDKVKEACSKHLKVAAYCTTQVERNACLFCKARKLDDKFYQKLRGQFPDAVFWQEIGEIFRQLQKQAAEIYNQSLIELYYEIFIKGKGFANASSVEHYLSDVCYTRAAELFKNAAIASGLRGKVKSNFRLKELKNMKSGLPTTKSDNFPIPLVKQKGGQYTGFEISSHNDDFIIKIPFGRWQVKKEIDKYRPWEKFDFEQVRKSPKPISLLLSTQRRKRNKGWSKDEGTEAEIRKVMNGDYQTSYIEVKRGSKTGEKSAWMLNLSIDVPKIDKGVDPSIIGGIDVGVKSPLVCAINNAFSRYSISDNDLFRFNKKMFARRRILLKKNRHKRAGHGAKNKLKPISILTEKSKRFRKKLIERWACEIADFFIRNKVGTVQMENLESMKGKEDSYFNIRLRGFWPYAEMQSKIEFKLKQYGIEIRKVAPNNTSRTCSKCGHLNNYFNFEYRKKNKFPHFKCEKCYFKEDADYNAALNISNPRLKSTKEEP

SEQ ID NO: 7 - protein, 726 aa, synthetic construct
SEVEFSHEYWMRHALTLAKRARDEREVPVGAILVLNNRVIGVGWNRAIGLHDPTAHAEIMALRQGGLVTQNYRLIDATLYVTFEPCVMCAGAMIHSRIGRVVFGVRNSKHGAAGSLVNVLNYPGMNHRVEITEGILADECAALLCDFYRMPRQVFNARKKAQSSINSGGSSGDSSGSETPGTSESATPKSSGGSSGGSAKNTITKALKLRIVRPYNSAEVEKIVADEKNNRERIALEKNKDKVKEACSKHLKVAAYCTTQVERNACLFCKARKLDDKFYQKLRGQFPDAVFWQEIGEIFRQLQKQAAEIYNQSLIELYYEIFIKGKGFANASSVEHYLSDVCYTRAAELFKNAAIASGLRGKVKSNFRLKELKNMRSGLPTTKSDNFPIPLVKQKGGQYTGFEISGHNDDFIIKIPFGRWQVKKEIDKYRPWEKFDFEQVRKSPKPISLLLSTQRRKRSKGWSKDEGTEAEIRKVMNGDYQTSYIEVKRGSKIGEKSAWMLNLSIDVPKIDKGVDPSIIGGIDVGVRSPLVCAINNAFSRYSISDNDLFRFNKKMFARRRILLKKNRHKRAGHGTKNKLKPITILTEKSGRFRKKLIERWACEIANFFIKNKVGTVQMENLESMKRKEDSYFNIRLRGFWPYAEMQNKIEFKLKQYGIKIRKVAPNNTSKTCSKCGHLNNYFSFEYRKKNKFPHFKCEKCNFKEDADYNAALNISNPKLKSTKEEP

SEQ ID NO: 8 - protein, 726 aa, synthetic construct
SEVEFSHEYWMRHALTLAKRARDEREVPVGAVLVLNNRAIGEGWNRAIGLHDPTAHAEIMALRQGGLVMQNYRLTDATLYVTFEPCVMCAGAMIHSRIGRVVFGVRNSKRGAAGSLMNVLNYPGMNHCVEITEGILVDECAALLCDFYRMPRQVLNAQKKAQSSISSGGSSGGSSGSETPGTSESATPESSGGSSGGSAKNTITKALKLRIVRPYNSAEVEKIVADEKDNRERIALEKNKGKVKEACSKHLKVAAYCTTQVERNACLFCKARKLDDKFYQKLRGQFPDAVFWQEIGEIFRQLQKQAAEIYNQSLIELYYEIFIKGKGFANASSVEHYLSDVCYTRAAELFKNAAIASGLRGKVKSNFRLKELKNMRSGLPTTKSDNFPIPLVKQKGGQYAGFEISSHNDDFIIKIPFGRWQVKKEIDKYRPWEKFDFEQVRKSPKPISLLLSTRRRKRNKGWSKDEGTEAEIRRVMNGDYQTSYIEVKRGSKIGEKGAWMLSLSIDVPKIDKGVDPRIIGGIDVGVKSPLVCAINNVLSRYSISDNDLFHFNKKMFARRRILLKKNGHKRAGHGAKNKLKPITIMTEKSKRFRKKLIERWACEIADFFIKNKVGTVQMENLESMKRKEDSYFNIRLRGFWPYAEMQNKIEFKLKQYGIVVRKVAPNNTSKTCSQCGHLNNYFNFEYRKKNKFPYFKCEKCNFKENADYNAALNISNPQLKSTKGEP

SEQ ID NO: 9 - protein, 726 aa, synthetic construct
SEVEFSHEYWMRHALTLAKRARDEREVPVGAVLVLDNRVIGVGWNRAIGLHDPTAHAEIMALRQGGLVMQNYRLTDATLYVTFEPCVMCAGAMVHSRIGRVVFGVRNSKRGAAGSLMNVLNYPGMSHCVEITEGILVDECAALLCDFYRMPRQVLNAQKKAQSSISSGGSSGGSGGGETPGASESVTPKSSGGSSAGSTKNTITKTLKLRIVRPYNSAEVEKIVADEKNSREKIALEKNKDKVKEACSEHLKVAAYCTTQVERSACLFCKARKLDDKFYQKLRGQFPDAVFWQELGGIFRQLQKQAAEIYNQSLIELYYEIFIKGKGITNASRVEHYLSDVCYTRAAELFKNAAIASGLRNKIKSNFRLKELRNMKSGLPTTKSDNFPIPLVRQKGGQYTGFEISNHNGDFIIKIPFGRWQVKKEISKHRPWEKFDFEQVRKSPKPISLLLSTQRRKRNKGWGKDEGTEAEIRKVMNGDYQTSYIEVKRGSKIGEKSAWMLNLSIDVPKIDKGVDPSIIGGIDVGVKSPLVCAINNALSRYSISDNDLFHFNKKMFARRRILLRKNRHKRAGHGARNKLKPITVLTEKSERFRKKLIERWACEIANFFIKNKVGTVQMENLESMKRREDSYFNIRLRGFWAYAEMQSKIEFKLKQYGIKIRKVAPNNTSKTCSKCGHLNNYFNFEFRKKNKFPHFKCEKCNFKEDADYNAALNISNPKLKSTKEEP

SEQ ID NO: 10 - protein, 726 aa, synthetic construct
SEVEFSHEYWMRHALTLAKRARDEREVPVGAVLVLNNRVIGEGWNRAIGLHDPTAHAEIMALRQGGLAMQNYRLVDATLYVTFEPCVLCAGAMVHSRIGRVVFGVRNSKRGAAGSLMNVLNHPGMNHRVEITGGILADECAALLCDFYRMPRQVFNARKKAQSSINSGGSSGGSSGSETPGTSESATPKNSGGSSGGSAKNTITKTLQLRIVRPYNSAEVEKIVTDEKNNREKIALEKNKDKVKEACSKHLKMASYCTTQVERNACLFCKARKLDDKFYQKLRGQFPDAVFWQELGGIFRQLQKQAAEIYNQSLIELYYEIFIKGKGITNASRVEHYLSDVCYTRAAELFKNAAIASGLRSKVRSNFRLKELKNMKSGLPTTKSDNFPIPLVKQKGGQYTGFEISSHNSDFIIKIPFGRWQVKEEIVKYRPWEKFDFEQVRKSPKPISLLLSTQRRKRNKGWSKDEGTEAEIRKVMNGDYQTSYIEVKRGSKIGEKSAWMLNLSIDVPKIDKGVDPSIVGGIDVGVKSPLVCAIDNALSRYSISDNDLFHFNKKMFARRRILLKKNRHRRAGHGAKNKLKPISILTEKSKRFRKKLIERWACEIADFFIKNKVGTVQMENLESMKRKEDSYFNIRLRGFWPYAEMQNKIEFKLKQYGIEIRKVAPNNTSKTCSKCGHLNNYFNFEYRKKNKFPHFKCEKCNFKENADYNAALNISNPMLKSTKEKP

SEQ ID NO: 11 - protein, 726 aa, synthetic construct
SEVEFSHEYWMRHALTLAKRARDEREVPVGAVLVLNNRVIGEGWNRTTGLHDPTAHAEIMALRQGGLVMRNYRLTDATLYVTFEPCVMCAGAMIHSRIGRVVFGARNSKRGAAGSLMNVLSYPGMNHRVEITEGILADECAALLCDFYRMPRRVFNAQKKAQSSINSGGSSGGGSGSETPSTSESTTPVSSSGSSGGSAKNTITKTLKLRIVRPYNSAEVEKIVADEKNNREKIALARNKDKVKEACSEHLKVAAYCTTQVERNACLFCKARKLDDKFYQKLRGQFPDAVFWQELGEILRQLQKQAAEIYNQSLIELYYEIFIKGKGFANASSVEHYLSDVCYTRAAELFKNAAIASGLRGKVKSNFRLKELRSMKSGLPTTKSDNFPIPLVKQKGGQYTGFEISSHNDDFIIKIPFGRWQEKKEINKYRPWEKFDFEQVRKSPKPISLLLSTQRRKRNKGWSKDEGTEAEIRKVMNGNYQTSYIEVKRGSKIGEKSAWMLSLSIDVPKIDKGVDPSIIGGIDVGVKSPLVCAINNAFCRYSISDNDLFHFNKKMFARRRILLKKSRHKRAGHGAKNKLKPISILTEKSKRFRKKLIERWACEIADFFIKNKVGTVQMENLEGMKRKEDSYFNIRLRGFWPYAEMQNKIEFKLKQYGIEIRKVAPNNTSKTCSKCGHLNNYFNFEYRKKNKFPHFKCEKCNFKENADYNAALNISNPKLKSTKEEP

SEQ ID NO: 12 - protein, 726 aa, synthetic construct
SEVEFSHEYWMRHALTLAKRARDEREVPVGAILVLNDRVIGEGWNRAIGLHDPTAHAEIMALRQGGLVTQNYRLIDATLYVTFEPCIMCAGAMIHSRIGRVVFGVRNSKRGAAGSLMNVLDYPGMNHRVEITEGILAGECAALLCDFYRMPRQVFNAQKKAQSNINPGGSSGGSSGSETPGTSESPTPESSGGSSGGSAKNTITKTLKLRIVRPYNSAEVEKIVADEKDNREKIALEKNKDKVKEACSEHLKVAAYCTTQVERNACLFCKARKLDDKFYQKLKGQFPDAVFWQEIGEIFRQLQKQAAEIYNQSLIELYYEIFIKGKGFANASSVEHYLSDVCYTRAAELFKNAAIASGLRGKVKSNFRLKELKNMKSGLPTTKSDNFPIPLVKQKGGQYTGFEISSHNDDFIIKIPFGRWQVKKEIDKYRPWEKFDFEQVRKSPKPISLLLSTQRRKRNRGWSKDEGTEAEIRKVMNGDYQTSYIEVKRGSKIGEKSAWMLNLSIDVPKIDKGVDPSIIGGIDVGVKSPLVCAINNAFSRYSISDNDLFRFNKKMFARRRILLGKNRHKRAGHGVKNKLKPITILTEKSGRFRKKLIERWACEIADFFVKNKVGTVQMENLESMKRKEDSYFNIRLRGFWPYAEMQNKIEFKLKQYGIKVRKVAPNNTSKTCSKCGHLNNYFSFEYRKKNKFPHFKCEKCNFKENADYNAALNISNPKLKSTKEEP

SEQ ID NO: 13 - protein, 726 aa, synthetic construct
SEVEFSHEHWMRHALTLAKRARDEREVPVGAVLVLNNRVIGEGWNRTTGLHDPTAHAEIMALRQGGLVMQNYRLIDATLYVTFEPCVMCAGAMIHSRIGRVVFGVRNNKHGAAGSLVNVLNYPGMNHRVEITEGILADECAALLCDFYRMPRQVFNARKKAQSSINPGGSPGGSSGSETPGASESVTPKSSGGSSAGSTKNTITKTLKLRIVRPYNSAEVEKIVADEKNNREKIALEKNKDKVKEACSKHLKVASYCTTQVERNACLFCKARKLDDKFYQKLRGQFPDAVFWQELGEILRQLQKQAAEIYNQSLIELYYEIFIKGRGFANAGSVEHYLSDVCYTRAAELFKNAAIASGLRGKVKSNFRLKELKNMKSGLPTTKSDNFPIPLVKQKGGQYTGFEISSHNDDFIIKIPFGRWQVKKEIDKYRPWEKFDFEQVRKSPKPISLLLSTQRRKRNKSWSKDEGTEAEIRKVMNGDYQTSYIEVKRGSKIGEKSAWMLNLSIDVPKIDKGVDPSIVGGIDVGVKSPLVCAIDNALSRYSISDNDLFHFNKKMFARRRILLKKNGHRRAGHGAKNKLKPISVLTEKSKRFRKKLIERWACEIADFFIKNKVGTVQMENLESMKRKEDSYFNIRLRGFWPYAEMQNKIEFKLKQYGIVVRKVAPNNTSKTCSKCGHLNNYFNFEYRKKNKFPHFKCEKCNFKENADYNAALNISNPKLKSTKGEP

SEQ ID NO: 14 - protein, 726 aa, synthetic construct
SEVEFSHEYWMRHALTLAKRARDEREVPVGAVLVLNNRVIGEGWNRAIGLHDPTAHAEIMALRQGGLVMQNYRLTDATLYVTFEPCVMCAGAMIHSRIGRVVFGVRNSKRGAAGSLMNVLNYPGMNHCVEITEGILVDECAALLCDFYRMPRQVLNAQKKAQSSISSGGSSGGSSGSVTPGASGSVTPKSSGGSSAGSTKDTITKTLKLRIVRPYNSAEVEKIVADEKNNREKIALEKNKDKVKEACSKHLKVASYCTTQVERNACPFCKARKLDDKFYQKLRGQFPDAVFWQELGEILRQLQKQAAEIYNQSLIELYYEIFIKGKGITNASRVEHYLSDVCYTRAAELFKNAAIASGLRNKIKSNFRLKELRNMKSGLPTTKSDNFPIPLVRQKGGQYTGFEISNHDGDFIIKIPFGRWQAKKEIDKYRPWEKFDFEQVRKSPKPISLLLSTQRRKRNKGWSKDEGTEAEIRKVMNGDYQTSYIEVKRGSKTGEKSAWMLNLSIDVPRIDKGVDPSIIGGIDVGVKSPLVCAINNAFSRYSISDNDLFRFNKKMFARRRILLRKNRHKRAGHGAKNKLKPITMMTEKSKRFRKKLIERWACEIADFFIKNKVGTVQMENLESMKRKEDSYFNIRLRGFWPYAEMQNKIEFKLKQYGIVVRKVAPNNTSKTCSKCGHLNNYFNFEYRKKNKFPHFKCEKCNFKEDADYNAALNISNPKLKSTKEEP

SEQ ID NO: 15 - protein, 726 aa, synthetic construct
SEVEFSHEYWMRHALTLAKRARDEREVPVGAVLVLNNRVIGEGWNRAIGLHDPTAHAEIMALRQGGLVMQNYRLTDATLYVTFEPCVMCAGAMIHSRIGRVVFGVRNGKRGAAGSLMNVLNYPGMNHCVEITEGILVDECAALLCDFYRMPRQVLNAQKKAQSSISPGDSSGGSSGSETPGASGSVAPKSSGGSSGSSAKNTITKTLKLRIVRPYNSAEVEKIVADEKNNREKIALEKNKGKVKEACSKHLKVASYCTTQVERNACPFCKARKLDDKFYQKLRGQFPDAVFWQELGEILRQLQKQAAEIYNQSLIELYYEIFIKGRGFANASSVEHYLSDVCYTRAAELFKNAAIASGLRGKVKSNFRLKELRNMKSGLPTTKSDNFPIPLVRQKGGQYTGFEISNHDGDFIIKIPFGRWQVKKEINKYRPWEKFDFEQVRKSPKPISLLLSTQRRKRNKGWSKDEGTEAEIRKVMNGDYQTSYIEVKRGSKIGEKSAWMLNLSIDVPKIDKGVDPSIIGGIDVGVKSPLVCAINNAFSRYSISDNDLFRFNKKMFARRRILLRKNRHKRAGHGAKNKLKPISILTGKSERFRKKLIERWACEIADFFIKNKVGTVQMENLESMKRKEDSYFNIRLRGFWPYAEMQNKIEFKLKQYGIEIRKVAPNNTSKTCSKCGHLNNYFNFEYRRKNKFPHFKCEKCNFKENADYNAALNISNPKLKSTKEEP

SEQ ID NO: 16 - protein, 726 aa, synthetic construct
SEVEFSHEYWMRHALTLAKRARDEREVPVGAILVLNNRVIGEGWNRAIGLHDPTAHAEVMALRQGGLVMQNYRLIDATLYVTFEPCVMCAGAMIHSRIGRVVFGVRNSKHGAAGSLVNVLNYPGMNHRIEITEGILADECAALLCDFYRMPRQVFNARKKAQSSINSGGSSGGSSGSETPGTSESATPKNSGGSSGGSAKNTITKTLKLRIVRPYNSAEVEKIVADEKNNREKIALEKNKDKVKEACSKHLKVASYCTTQVERNACLFCKARKLDDKFYQKLRGQFPDAVFWQELGEIFRQLQKQAAEIYNQSLIELYYEIFIKGKGFANASSVEHYLSDVCYTRAAELFKNAAIASGLRGKVKSNFRLKELKNMKSGLPTTKSDNFPIPLVRQKGGQYTGFEISSHNDDFIIKIPFGRRQVKKEINKYRPWEKFDFEQVRKSPKPISLLLSTQRRKRNKGWGKDEGTEAEIRKVMNGDYQTSYIEVKRGSKIGEKSAWMLNLSIDVPKIDKGVDPSIIGGIDVGVKSPLVCAINNAFSRYSISDNDLFRFNKKMFARRRILLKKNKHKRAGHGAKNKLKPISILTGKSERFRKKLIERWACEIADFFIKNKVGTVQMENLESMKRKEDSYFNIRLRGFWPYAEMQSKIEFKLKQYGIEIRKVAPNNTSKTCSKCGHLNNYFSFEYRKKNKFPHFKCEKCSFKEDADYNAALNISNPKLKSTKEEP

SEQ ID NO: 17 - protein, 726 aa, synthetic construct; identical to SEQ ID NO: 10

SEQ ID NO: 18 - protein, 726 aa, synthetic construct
SEVEFSHEYWMRHALTLAKRARDEREVPVGAVLVLNNRVIGEGWNRAIGLHDPTAHAEIMALRQGGLVMQNYRLIDATLYVTFEPCVMCAGAMIHSRIGRVVFGVRNNKHGAAGSLVNVLDYPGMNHRVEITEGILADECAALLCDFYRMPRQVFNARKKARSSINSGGSSGGSSGSVTPGPSESATPESSGGSSGSSAKSTITKTLQLRIVRPYNSAEVEKIVADEKNNREKIALEKNKDKVKEACSKHLKVASYCTTQVERNACLFCKARKLDDKFYQRLRGQFPDAVFWQELGEIFRQLQKQAAEIYNQSLIELYYEIFIKGKGFANASSVEHYLSDVCYTRAAELFKNAAIASGLRGKVKSNFRLKELKNMKSGLPTTKSDNFPIPLVRQKGGQYTGFEISSHNDDFIIKIPFGRWQVRKEIDKYRPWEKFDFEQVRKSPKPISLLLSTQRRKRNKGWSKDEGTEAEIRKVMNGDYQTSYIEVKRGSKTGEKSAWMLNLSIDVPKIDKGVDPSVIGGIDVGVKSPLVCAINNAFSRYSISDNDLFRFNKKMFARRRILLKKNRHKRAGHGAKNKLKPISILTEKSKRFRKKLIERWACEIADFFIKNKVGTVQMENLESMKRKEDGYFNIRLRGFWPYAEMQNKIEFKLKQYGIEIRKVAPNNTSKTCSKCGHLNNYFNFEYRKTNKFPHFKCEKCNFKEDADYNAALNISNPKLKSTKEEP

SEQ ID NO: 19 - protein, 726 aa, synthetic construct
SEVEFSHEYWMRHALTLAKRARDEREVPVGAVLVLNNRVIGEGWNRAIGLHDPTAHAEIMALRQGGLVMQNYRLIDATLYVTFEPCVMCAGAMIHSRIGRVVFGVRNSKHGAAGSLVNVLNYPGMNHRVEITEGILVDECAALLCDFYRMPRQVLNAQKKAQSSISSGGSSGGSSGSVTPGASGSVTPKSSGGSSAGSTKDTITKTLKLRIVRPYNSAEVEKIVADEKNNREKIAMEKNKDKVKEACSKHLKVASYCTTQVERNACLFCKARKLDDKFYQELRGQFPDAVFWQELGGIFRQLQKQAAEIYNQSLIELYYEIFIKGKGITNASRVEHYLSDVCYTRAAELFKNAAIASGLRSKVRSNFRLKELKNMKSGLPTTKSDNFPIPLVKQKGGQYTGFEISSHNDDFIIKIPFGRWQAKKEIDKYRPWEKFDFEQVRKSPKPISLLLSTQRRKRNRGWSKDEGTEAEIRKVMNGDYQTSYIEVKRGSKIGEKSAWMLNLSIDVPKIDKGVDPSIIGGIDVGVKSPLVCAINNAFSRYSISDNDLFRFNKKMFARRRILLGKNRHKRAGHGVKNKLKPITILTEKSGRFRKKLIERWACEIADFFVKNKVGTVQMENLESMKRKEDSYFNIRLRGFWPYAEMQSKIEFKLKQYGIEIRKVAPNNTSKTCSKCGHLNNYFNFEYRKKNKFPHFKCEKCNFKENADYNAALNISNPKLKSTKEEP

SEQ ID NO: 20 - protein, 726 aa, synthetic construct
SEVEFSHEYWMRHALTLAKRARDEREVPVGAILVLNNRVIGEGWNRAIGLHDPTAHAEIMALRQGGLVMQNYRLIDATLYVTFEPCVMCAGAMIHSRIGRVVFGVRNNKHGAAGSLVNVLNYPGMNHRVEITEGILADECAALLCDFYRMPRQVFNARKKAQSSINPGGSSGGSSGSETPGTSESATPESSGGSSGSSAKNTITKTLKLRIVRPYNSAEVEKIVADEKNNREKIALEKNKDKVKEACSEHLKVVAYCTTQVERNACLFCKARRLDDKFYQKLRGQFPDAVFWQEIGEIFRQLQKQAAEIYNQSLIELYYEIFIKGKGFANASSMEHYLSDVCYTRAAELFKNAAIASGLRGKVKSNFRLKELKNMKSGLPTTKSDNFPIPLVKQKGGQYTGFEISNHNSDFIIKIPFGRWQVKKEINKYRPWEKFDFEQVRKSPKPISLLLSTQRRKRNKGWSKDEGTEAEIRKVMNGDYQTSYIEVKRGSRIGEKSAWMLSLSIDVPKIDRGVDPSIIGGIDVGVKSPLVCAINNALGRYSISDNDLFHFNKKMFARRRILLKKNRHKRAGHGAKNKLKPITILTEKSRRFRKKLIERWACEIADFFIKNKVGTVQMENLESMKRREDSYFNIRLRGFWPYAEMQNKIEFKLKQYGIEIRKVAPNNTSKTCSKCGHLNNYFNFEYRKKNKFPHFKCEKCNFKENADYNAALNISNPKLKGTKEEP

SEQ ID NO: 21 - protein, 726 aa, synthetic construct
SEVEFSHEYWMRHALALAKRARDAREVPVGAILVLNNRVIGEGWNRAIGQHDPTAHAEIMALRQGGLVMQNYRLIDATLYVTFEPCVMCAGAMIHSRIGRVVFGVRNSKHGAAGSLMNVLNYPGMNHRVEITEGILADECAALLCDFYRMPRQVFNGRKKAQSSINSGGSSGGSSGSEAPGTSESATPGSSGGSSGGSAKNTITKTLKLRIVRPYNSAEVEKIVADEKNNREKTALEKNKDKVKEACSEHLKVAAYCTTQVERSACLFCKARKLDDKFYQKLRGQFPDAVFWQEIGEIFRQLQKQAAEIYNQSLIELYYEIFIKGKGFANASSVEHYLSDVCYTRAAELFKNAAIASGLRGKVKSNFRLKELKNMKSGLPTTKSDNFPIPLVRQKGGQYTGFEISSHNDDFIIKIPFGRWQVKKEIDKYRPWEKFDFEQVRKSPKPISLLLSTQRRKRNKGWSKDEGTEAEIKKVMSGDYQTSYIEVKRGSKIGEKSAWMLSLSIDVPKIDRGVDPSIIGGIDVGVRSPLVCAINNASSRLSISDNDLFRFNKKMFARRRILLKKNGHKRAGHGAKNKLKPITVLTEKSVRFRKKLIERWACEIADFFIRNKVGTVQMENLESMKRKEDSYFNIRLRGFWPYAEMQNKIEFKLKQYGIVVRKVAPNNTSKTCSQCGHLNNYFNFEYRKKNKFPYFKCEKCNFKENADYNAALNISNPQLKGTKGEP

SEQ ID NO: 22 - protein, 726 aa, synthetic construct
SEVEFSHEYWMRHALTLAKRARDEREVPVGAVLVLNNRVIGEGWNRAIGLHDPTAHAEIMALRQGGLVMQNYRLADATLYVTFEPCVMCAGAMIHSRIGRVVFGVRNSKRGAAGSLMNVLNYPGMNHCVEITEGILVDECAALLCDFYRMPRQVLNAQKKAQSSISSGGSSGGSSGSETPGTSESATPESSGGSSGGSAKNTITKTLKLRIVRPYNSAEVEKIVADEKNNREKIALEKNKDKVKEACSKHLKVAAYCTTQVERNACLFCKARRLDDKFYQKLRGQFPDAVFWQEIGEIFRQLQKQAAEIYNQSLIELYYEIFIKGKGFANASSVEHYLSDVCYTRAAELFKNAAIASGLRGKVKSNFRLKELKNMKSGLPTTKSDNFPIPLVKQKGGQYTGFEISSHNDDFIIKIPFGRWQVKKEIDKYRPWEKFDFEQVRKSPKPISLLLSTQRRKRNKGWSKDEGTEAEIRKVMNGDYQTSYIEVKRGSKIGEKSAWMLNLSIDVPKIDKGVDPSIIGGIDVGVKSPLVCAINNAFSRYSISDNDLFRFNKKMFARRRILLKKNRHKRAGHGAKNKLKPISILTGKSERFRKKLIERWACEIADFFIKNKVGTVQMENLESMKRKEDSYFNIRLRGFWPYAEMQNKIEFKLKQYGIEIRKVAPNNTSKTCSKCGHLNNYFNFEYRKKSKFPHFKCEKCNFREDADYNAALNISNPKLKSTKEEP

SEQ ID NO: 23 - protein, 726 aa, synthetic construct
SEVEFSHEYWMRHALTLAKRARDEREVPVGAVLVLNNRVIGEGWNRAIGQHDPTAHAEIMALRQGGLVMQNYRLTDATLYVTFEPCVMCAGAMIHSRIGRVVFGVRNGKRGAAGSLMNVLNYPGMNHCVEITEGILVDECAALLCDFYRMPRQVLNAQKKAQSSISSGGSSGGSSGSETPGASESVTPKSSGGSSAGSTKNTITKTLKLRIVRPYNSAEVEKIVADEKNSREKIALERSKDKVKEACSEHLKVAAYCTTRVERNACLFCKARKLDDRFYQKLRGQFPDAVFWQETGEIFRQLQRQAAEIYNQSLIELYYEIFIKSKGFANASSVEHYLSDVCYTRAAELFKNAAIASGLRGKVKSNFRLKELKNMKSGLPTTKSDNFPIPLVKQKGGQYTGFEISSHNDDFIIKIPFGRWQVKKEIDKYRPWEKFDFEQVRKSPKPISLLLSTQRRKRNKGWSKDEGTEAEIRKVMNGDYQTSYIEVKRGSKTGEKSAWMLNLSIDVPKIDKGVDPSIIGGIDVGVKSPLVCAINNAFSRYSISDNDLFRFNKKMFARRRILLGKNRHKRAGHGVKNKLKPITILTEKSGRFRKKLIERWACEIADFFVKNKVGTVQMENLESMKRKEDSYFNIRLRGFWPYAEMQNKIEFKLKQYGIKVRKVAPNNTSKTCSKCGHLNNYFSFEYRKKNKFPHFKCEKCNFKENADYNAALNISNPKLKSTKEEP

SEQ ID NO: 24 - protein, 726 aa, synthetic construct
SEVEFSHEYWMRHALTLAKRARDEREVPVGAILVLNNRVIGVGWNRAIGLHDPTAHAEIMALRQGGLVTQNYRLIDATLYVTFEPCVMCAGAMIHSRIGRVVFGVRNSKRGAAGSLMNVLNYPGMNHRVEITEGILADECAALLCDFYRMPRQVFNARKKARSNINSGGSSGGSSGSETPGTSESATPESSGGSSGGSAKNTITKTLTLRIVRPYNSAEVEKIVADEKNNREKIALEKNKDKVKEACSEHLKVAAYCTTQVERNACLFCKARKLDDKFYQKLRGQFPDAVFWQEIGEIFRQLQKQAAEIYNQSLIELYYEIFIKGKGFANASSVEHYLSGVCYTRAAELFKNAAIASGLRGKVKSNFRLKELRNMKSGLPTTKSDNFPIPLVRQKGGQYTGFEISSHNDDFIIKIPFGRWQVKKEIDKYRPWEKFDFEQVRKSPKPISLLLSTQRRKRNKGWSKDEGTEAEIRKVMNGDYQTSYIEVKRGSKTGEKSAWMLNLSIDVPKIDKGVDPSIIGGIDVGVKSPLVCAINNALSRYSISDNDLFHFNKKMFARRRILLRKNRHKRAGHGARNKLKPITVLTEKSERFRKKLIERWACEIANFFIKNKVGTVQMENLGSMKRREDSYFNIRLRGFWPYAEMQSKIEFKLKQYGIEVRKVAPNNTSKTCSKCGHLNNYFNFEFRKKNKFPHFKCEKCNFKEDADYNAALNISNPKLKSTKEEP

SEQ ID NO: 25 - protein, 726 aa, synthetic construct
SEVEFSHEYWMRHALTLAKRARDEREVPVGAILVLNNRVIGEGWNRAIGLHDPTAHAEIMALRQGGLVLQNYRLIDATLYVTFEPCVMCAGAMIHSRIGRVVFGVRNSKHGAAGSLVNVLDYPGMNHRVEITEGVLADECAALLCDFYRMPRQVFNARKKAQSNINPGGSSGGSSGSETPGTSDSATPGSSGGSSGGSAKNTITKTLKLRIVRPYNSAEVEKIVADEKNNREKTALEKNKDKVKEACSEHLKVATYCTTQVERNACLFCKARKLDDKFYQKLRGQFPDAVFWQEIGEIFRQLQKQAAEIYNQSLIELYYEIFIKGKGFANASSVEHYLSDVCYTRAAELFKNAAIASGLRGKVKSNFRLKELKNMKSGLPTTKSDNFPIPLVKQKGGKYTGFEISSHNDDFIIKIPFGRWQVKEEIDKYRPWEKFDFEQVRKSPKPISLLLSTQRRKRNKGWSKDEGTEAEIRKVMNGDYQTSYIEVKRGSKIGEKSAWMLNLSIDVPKIDKGVDPSIIGGIDVGVKSPLVCAINNAFSRYSISDNDLFHFNKKMFARRRILLKKNRHKRAGHGAKNKLKPISILTEKSKRFRKKLIERWACEIANFFIKNKVGTVQMENLESMRRKEDSYFNIRLRGFWPYAEMQNKIEFKLKQYGIEIRKVAPNNTSKTCSKCGHLNNYFNFEYRKKNKFPHFKCEKCNFKENADYNAALNISNPKLKSTKEEP

SEQ ID NO: 26 - protein, 726 aa, synthetic construct
SEVEFSHEHWMRHALTLAKRARDEREVPVGAVLVLNNRVIGVGWNRAVGLHDPTAHAEIMALRQGGLVMQNYRLTDATLYVTFEPCVMCAGAMIHSRIGRVVFGVRNSKRGAAGSLMNVLNYPGMNHCVEITEGILMDECAALLCDFYRMPRQVLSAQKKAQSSISSGGPSGGSSCSETPGASESVTPKNSGGSSTGSTKNTITKTLKLRIVRPYNSAEVEKIVADEKNSREKIALEKNKDKVKEACSEHLKVAAYCTTQVERNACLFCKARKLDDRFYQKLRGQFPDAVFWQEIGEIFRQLQKQAAEIYNQSLIELYYEIFIKGKGIANASSVEHYLSDVCYTRAAELFKNAAIASGLRNKVKSNFRLKELRSMKSGLPTTKSDNFPIPLVKQKGGQYTGFEISSHNDDFIIKIPFGRWQVKKEIDKYRPWEKFDFEQVRKSPKPISLLLSTQRRRRNKGWGKDEGTEAEIRKVMSGDYQTSYIEVKRGSKVGEKSAWMLNLSIDVPKIDKGVDPSIIGGIDVGVKSPLVCAINNAFSRYSISDNDLYRFNKKMFARRRILLKKSKHKRAGHGAKNKLKPITILTEKSGRFRKKLIERWACEIADFFIKNKVGTVQMENLEGMKRKEDSYFNIRLRGFWPYAEMQNKIEFKLKQYGIEIRKVAPNNTSKTCSKCGHLNNYFNFEYRKKNKFPHFKCEKCNFKEDADYNAALNISNPKLKSTKEEP

SEQ ID NO: 27 - protein, 726 aa, synthetic construct
SEVEFSHEYWMRHALTLARRARDEREVPVGAVLVLNNRVIGEGWNRAIGLHDPTAHAEIMALRQGGLVMQNHRLTDATLYVTFEPCVMCAGAMIHSRIGRVVFGVRNSKRGAAGSLMNVLNYPGMNHCVEITEGILVDECAALLCDFYRMPRQVLNAQKKAQSSISSSGSSGGSSGSVTPGTSESPTPESSGGSPGGSAKNTITKTLKLRIVRPYNSAEVEKIVADEKNNREKIALEKNKGKVKEACSKHLKVATYCTTQVERNACLFCKARKLDDKFYQKLRGQFPDAVFWQELGEILRQLQKQAAEIYNQSLIELYYEIFIKGRGFANASSVEHYLSDVCYTRAAELFKNAAIASGLRGKVKSNFRPKELKNMKSGLPTTKSDNFPIPLVKQKGGQYTGFEISSHNDDFIIKIPFGRWQVKKEIDKYRPWEKFDFEQVRKSPKPISLLLSTQRRKRNKGWSKDEGTEAEIRKVMNGDYQTSYIEVKRGSKIGEKSAWMLSLSIDVPKIDKGVDPSIIGGIDVGVKSPLVCAINNSFSRYSICDNDLFRFNKKMFARRRILLKKSKHKRAGHGAKNKLKPITTMTEKSKRFRKKLIERWACEIADFFIKNRVGTVQMENLESMKRKEDSYFNIRLRGFWPYAEMQNKIEFKLKQYGIEIRKVAPNNTSKTCSKCGHLNNYFNFEYRKKNKFPYFKCEKCNFKENADYNAALNISNPKLKGTKEEP

SEQ ID NO: 28 - protein, 726 aa, synthetic construct
SEVEFSHEYWMRHALTLAKRARDEREVPVGAILVLNNRVIGEGWNRAIGLHDPTAHAEVMALRQGGLVMQNYRLTDATLYVTFEPCVMCAGAMIHSRIGRVVFGVRNSKHGAAGSLVNVLNYPGMNHRVEITEGILADECAALLCDFYRMPRQVFNARKKAQSSINSGGSSGGSSGSETPGTSESATPKSSGGSSGGSAKNTITKALKLRIVRPYNSAEVEKIVADEKNNRERIALEKNKDKVKEACSEHLKVAAYCTTQVERSACLFCKARKLDDKFYQKLRGQFPDAVFWQEIGEIFRQLQKQAAEIYNQSLIELYYEIFIKGKGFANASSVEHYLSDVCYTRAAELFKNAAIASGLRGKVKSNFRLKELKNMKSGLPTTKSDNFPIPLVKQKGGQYTGFEISSHNSDFIIKIPFGRWRVKEEIDKYRPWEKFDFEQVRKSPKPISLLLSTQRRKRNKGWSKDEGTEAEIRKVMNGDYQTSYIEVKRGSKIGEKSTWMLSLSIDVPKIDKGVDPSIIGGIDVGVRSPLVCAIDNAFSRYSISDNDLFHFNKKMFARRRILLKKNRHKRAGHGAKNKLKPISILTEKSKRFRKKLIERWACEIADFFIKNKVGTVQMENLESMKRKEDSYFNIRLRGLWPYAEMQNKIEFKLKQYGIKIRRVAPNNTSKTCSKCGHLNNYFSFEYRKKNKFPHFKCEKCNFKENADYNAALNISNPKLMSTKEEP

SEQ ID NO: 29 - protein, 726 aa, synthetic construct
SEVEFSHEYWMRHALTLAKRARDEREVPVGAVLVLNNRVIGEGWNRAIGLHDPTAHAEIMALRQGGLVMQNYRLTDATLYVTFEPCVMCAGAMIHSRIGRVVFGVRNSKRGAAGSLMNVLNYPGMNHCVEITEGILVDECAALLCDFYRMPRQVLNAQKKAQSSINSGGSSGGSSGSETPGTSGSATPGSSGGGSSGSAKNTITKTLQLRIVRPYNSAEVEKIVADEKNNREKIALEKNKDKVKEACSKHLKVASYCTTQVERNACPFCKARKLDDKFYQKLRGQFPDAVFWQELGEIFRQLQKQAAEIYNQSLIELYYEIFIKGKGITNASRVEHYLSDVCYTRAAELFKNAAIASGLRSKVRSNFRLKELKNMKSGLPTTKSDNFPIPLVKQKGGQYTGFEISSHNSDLIIKIPFGRWQVKEEIDKYRPWEKFDFEQVRKSPKPISLLLSTQRRQKNKGWSKDEGTEAEIRRVMNGDYQTSYIEVKRGSKIGEKSTWMLNLSIDVPKIDKGVDPSIVGGIDVGVKSPLVCAINNSFSRYSICDNDLYRFNKKMFARRRILLKKNRHKRAGHGAKNKLKPISILTEKSKRFRKKLIERWACEIADFFIKNKVGTVQMENLESMKRKEDSYFNIRLRGFWPYAEMQNKIEFKLKQYGIVVRKVAPNNTSKTCSKCGHLNNYFNFEFRKKNKFPHFKCEKCNFKEDADYNAALNISNPKLKSTREEP

SEQ ID NO: 30 - protein, 726 aa, synthetic construct
SEVEFSHEHWMRHALTLAKRARDEREVPVGAVLVLNNRVIGEGWNRAIGLHDPTAHAEIMALRQGGLVMQNYRLTDATLYVTFEPCVMCAGAMIHSRIGRVVFGVRNSKRGAAGSLMNVLNYPGMNHCVEITEGILVDECAALLCDFYRMPRQVLNAQKKAQSSISPGGLSGGSSGSETPGASESVTPKSSGGSSGGSAKNTITKTLKLRIVRPYNSAEVEKIVADEKNNREKIALEKNKGKVKEACSKHLEVAAYCTTQVERNACLFCKARKLDDKFYQKLRGQFPDAVFWQELGEIFRQLQKQAAEIYNQSLIELYYEIFIKGKGFANASSVEHYLSDVCYTRAAELFKNAAIASGLRNKIKSNFRLKELRNMKSGLPTTKSDNFPIPLVRQKGGQYTGFEISNHDGDFIIKIPFGRWQVKKEINKHRPWEKFDFEQVRKSPKPISLLLSTQRRKRNKGWSKDEGTEAEIRRVMNGDYQTSYIEVKRGSKIGEKSAWMLNLSIDVPKIDKGVDPSIIGGIDVGVKSPLVCAINNALSRYSISDNDLFHFNKKMFARRRILLRKNRHKRAGHGAKNKLKPITIMTEKSKRFRKKLIERWACEIADFFIKNKVGTVQMENLESMKRKEDSYFNIRLRGFWPYAEMQSKIEFKLKQYGIVVRRVAPNNTSKTCSKCGHLNNYFNFEYRKKNKFPHFKCERCNFKENADYNAALNISNPKLKSTKEEP

SEQ ID NO: 31 - protein, 726 aa, synthetic construct
SEVEFSHEYWMRHALTLAKRARDEREVPVGAVLVLNNRVIGEGWNRAIGLHDPTAHAEIMALRQGGLVMQNYRLVDATLYVTFEPCVMCAGAMIHSRIGRVVFGVRNNKHGAAGSLVNILNYPGMNHRVEITEGILVDECAALLCDFYRMPRQVLNARKKAQSSINSGGSSGGSNGSVTPGTSESATPESSGGSFGGSAKNTVTKTLQLRIVRPYNSAEVEKIVADEKNSREKIALEKNKDKVKEACGKHLKVASYCTTQVERNACLFCKARKLDDKFYQKLRGQFPDAVFWQELGEIFRQLQKQAAEIYNQSLIELYYEIFIKGKGFANASSVEHYLSDVCYTRAAELFKNAAIASGLRGKVKSNFRLKELKNMKSGLPTTKSDNFPVPLVKQKGGQYTGFEISSHNDDFIIKIPFGRWQVKKEIDKYRPWEKFDFEQVRKSPKPISLLLSTQRRKRNKGWSKDEGTEAEIKKVMNGDYQTSYIEVKRGSKIGEKSAWMLSLSIDVPKIDKGVDPSIIGGIDVGVRSPLVCAINNAFSRYSISDNDLFRFNKKMFARRRILLKKNRHKRAGHGAKNKLKPITILTEKSRRFRKKLIERWACEIADFFIKNKVGTVQMESLESMKRKEDSYFNIRLRGFWPYAEMQNKIEFKLKQYGIEVRKVAPNNTSRTCSKCGHLNHYFNFEYRKKNKFPHFKCEKCNFKENADYNAALNISNPKLKSTKGEP

SEQ ID NO: 32 - protein, 726 aa, synthetic construct
SEVEFSHEYWMRHALTLAKRARDKHEVPVGAVLVLDNRVIGEGWNRTTGLHDPTAHAEIMALRQGGLVMRNYRLTDATLYVTFEPCVMCAGAMIHSRIGRVVFGVRNSKRGAAGSLMNVLNYPGMNHCVEITEGILVDECAALLCDFYRMPRQVLNAQKKAQSSISPGGSSGGSSGSETPGASESVTLKSSGGSSGGSVKNTITKTLKLRIVRPYNSAEVEKIVADEKNNREKIALEKNKGKVKEACSRHLEVAAYCTTQVERNACLFCKARKLDDKFYRKLRGQFPDAVFWQELGEIFRQLQKQAAEIYNQSLIELYYEIFIKGKGFANASSVEHYLSDVCYTRAAELFKNAAIASGLRGKVKSNFRLKELKNMKSGLPTTKSDNFPIPLVKQKGGQYTGFEISSHNDDFVIKIPFGRWQVKKEIDKYRPWEKFDFEQVRKGPKPISLLLSTQRRKRNKGWSKDEGTEAEIRKVMSGDYQTSYIEVKRGSKTGEKSAWMLNLSIDVPKIDKGVDPSIIGGIDVGVKSPLVCAINNALSRYSISDNDLFHFNKKMFARRRILLKKNRHKRAGHGAKNKLKPISILTEKSERFRKKLIERWACEIADFFIKNKVGTVQMENLESMKRREDSYFNIRLRGFWPYAKMLNKIEFKLKQYGIKIRKVAPNNTSKTCSKCGHLNNYFNFEYRKKNKFPHFKCEKCNFKENADYNAALNISNPKLKSTKGES

SEQ ID NO: 33 - protein, 726 aa, synthetic construct
SEVEFSHEYWMRHALTLAKRARDEREVPVGAILVLNNRVIGEGWNRAISLHDPTAHAEIMALRQGGLVMQNYRLIDATLYVTFEPCVMCAGAMIHSRIGRVVFGVRNNKHGAAGSLVNVLNYPGMNHRVEITEGILADECAALLCDFYRMPRQVFNARKKAQSSINPGGSSGGSSGSETPGTSESATPESSGGSSGSSAKNTITKTLKLRIVRPYNSAEVEKIVADEKNNREKIALEKNKDKVKEACSKHLKVAAYCTTQVERNACLFCRARKLDDKFYQKLRGQFPDAVFWQETSEIFRQLQKQAAEIYNQSLIELYYEIFIKGKGFANASSVEHYLSDVCYTRAAGLFKNAAIASGLRGKVKSNFRLKELKNMKSGLPTTKSDNFPIPLVKQKGGQYTGFEISSHNDDFIIKIPFGRWQVKKEIDKYRPWEKFDFEQVRKSPKPISLLLSTQRRRRNKGWSKDGGTEAEIRKVMNGDYQISYIEVKRGNKIGEKSAWMLNLSIDVPKIDKGVDPSIIGGIDVGVKSPLVCAINNALSRYSISDNDLFRFNKKMFARRRILLKKNGHKRAGHGAKNKLKPITIMTEKSKRFRKKLIERWACEIADFFIKNKVGTVQMENLESMKRKEDSYFNIRLRGFWPYAEMQNKIEFKLKQYGIKIRKVAPNNTSKTCSKCGHLNNYFNFEYRKMNKFPHFKCEKCNFKEDADYNAALNISNPKLKSTKEEP

SEQ ID NO: 34 - protein, 726 aa, synthetic construct
SEVEFSHEYWMRHALTLAKRARDEREVPVGAVLVLNNRVIGEGWNRAIGLHDPTAHAEIMALRQGGLVMQNYRLTDATLYVTFEPCVMCAGAMVHSRIGRVVFGVRNSKRGAAGSLMNVLNYPDMNHCVEITEGILVDECAALLCDFYRMPRQVLNSQKKAQSSISSGGSSGGSSGSETPGASESATPKSSGGSSGGSTKNTITKTLKLRIVRPYNSAEVEKIVADEKNNREKIALEKNKGKVKEACSKHLEVAAYCTTQVERNACLFCKARKLDDKFYQKLRGQFPDAVFWQELGEIFRQLQKQAAEIYNQSLIELYYEIFIKGKGFANASSVEHYLSDVCYTRAAELFKNAAIASGLRGKVKSNFRLKELKNMKSGLPTTKSDNFPIPLVKQKGGQYTGFEISSHNDDFIIKIPFGRWQVRKEIDKYRPWEKFNFEQVRKGPKPISLLLSTQRRKRNKGWSKDEGTEAEIRKVMNGDYQTSYIEVKRGSKIGEKSAWMLSLSIDVPKIDKGVDPSIIGGIDVGVKSPLVCAINNAFSRYSISDNDLFRFNKKMFARRRILLGKNRHKRAGHGVKNKLKPITILTEKSGRFRKKLIERWACEIADFFVKNKVGTVQMENLESMKRKEDSYFNIRLRGFWPYAEMQDKIEFKLKQYGIKVRKVAPNNTSKTCSKCGHLNNYFNFEYRRKNKFPHFKCEKCNFKEDADYNAALNISNPKLKSTMEEP

SEQ ID NO: 35 - protein, 726 aa, synthetic construct
SEVEFSHEYWMRHALTLAKRARDEREVPVGAVLVLNNRVIGVGWNRAIGLHDPTAHAEIMALRQGGLVTQNYRLIDATLYVTFEPCVMCAGAMIHSRIGRVVFGVRNNKHGAAGSLVNVLNYPGMNHRVEITEGVLADECAALLCDFYRMPRQVFNARKKAQSSINPGGPSGGSSGSKTPGTSESATPEGSGGGSSGSAKNTITKTLQLKIVRPYNSAEVEKIVADEKNNREKIALEKNKDKVKEACSKHLKVASYCTTQVERSACPFCKARKLDDKFYQKLGGQFPDAVFWQELGEILRQLQKQAAEIYNQSLIELYYEIFIKGRGFANASSVEHYLSDVCYTRAAELFKNAAIASGLRGKVKSNFRLKELKNMKSGLPTTKSDNFPIPLVKQKGGQYTGFEISSHNDDFIIKIPFGRWQVKKEIDKYRPWEKFDFEQVRKSPKPISLLLSTQRRKRNKGWSKDEGTEAEIRKVMNGDYQTSYIEVKRGSKTGEKSAWMLNLSIDVPKIDKGVDPSIIGGIDVGVKSPLVCAINNALSRYSISDNDLFRFNKKMFARRRILLKKNRHKRAGHGAKNKLKPITILTEKSKRFRKKLIERWACEIADFFVKNKVGTVQMENLESMKRKEDSYFNIRLRGFWPYAEMQNKIEFKLKQYGIEIRKVAPNNTSKTCSKCGHLNNYFNFEYRKKNKFPHFKCEKCNFKENADYNAALNICNPKLKSTKEEP

SEQ ID NO: 36 - protein, 726 aa, synthetic construct
SEVEFSHEYWMRHALTLAKRARDEREVPVGAILVLNNRVIGEGWNRAIGLHDPTAHAEIMALRQGGLVMQNYRLTDATLYVTFEPCVMCAGAMIHSRIGRVVFGVRNSKRGAAGSLMNVLNYPGMNHCVEITEGILVDECAALLCDFYRMPRQVLNAQKKAQSSISSGGSSGGSSGNETPGASESATPKSSSGSSAGSTKNTITKTLKLRIVRPYNSAEVEKIVADEKNNRERIALEKNKDKVKEACSKHLKVAAYCTTQVERNACLFCKARKLDDKFYQKLRGQFPDAVFWQETGEIFRQLQRQAAEIYNQSLIELYYEIFIKGKGIANASSVEHYLSDVCYTRAAELFKNAAIASGLRNKIKSNFRLKELRNMKSGLPTTKSDNFPIPLVRQKGGQYTGFEISNHNGDFIIKIPFGRWQVKKEIDKYRPWEKFDFEQVRKSPKPISLLLSTQRRKRNRGWSKDEGTEAEIRKVMNGDYQTSYIEVKRGSKIGEKSAWMLNLSIDVPKIDKGVDPSIIGGIDVGVKSPLVCAINNAFSRYSISDNDLFRFNKKMFARRRILLGKNRHKRAGHGVKNKLKPITILTEKSGRFRKKLIERWACEIADFFVKNKVGTVQMENLESMKRKEDSYFNIRLRGFWPYAEMQNKIEFKLKQYGIKVRKVAPNNTSKTCSKCGHLNNYFSFEYRKKNKFPHFKCEKCNFKEDADYNAALNISNPKLKSTKEEP

SEQ ID NO: 37 - protein, 726 aa, synthetic construct
SEVEFSHEYWMRHALTLAKRARDEREVPVGAVLVLNNRVIGEGWNRAIGLHDPTAHAEIMALRQGGLVMQNYRLIDATLYVTFEPCVMCAGAMIHSRIGRVVFGVRNNKHGAAGSLVNVLNYPGMNHRVEITEGILADECAALLCDFYRMPRQVFNARKKVRSSINPGGSSGGSSGGDTLGASESVTPKSSVGSSASSTKNTITKTLKLRIVRPYNSAEVEKIVADEKDNREKIALEKNKDKVKEACSKHLKVAAYCTTQVERNACLFCKARKLDDKFYQKLRGQFPDAVFWQELGEILRQLQKQAAEIYNQSLIELYYEIFIKGRGFANASSVEHYLSDVCYTRAAELFKNAAIASGLRGKVKSNFRLKELKNMKSGLPTTKSDNFPIPLVKQKGGQYTGFEISSHNDDFIIKIPFGRWQVKKEIDKYRPWEKFDFEQVRKSPKPISLLLSTQRRKRNKGWSKDEGTEAEIRKVMNGDYQTSYIEVKRGSKIGEKSAWMLNLSIDVPKIDKGVDPSIIGGIDVGVKSPLVCAINDAFSRYSISDNDLFRFNKKVFARRRILLKKNRHKRAGHGTKNKLKPITILTEKSGRFRKKLIERWACEIADFFIKNKVGTVQMENLESMKRREDSYFNIRLRGFWPYAEMQNKIEFKLKQYGIKIRKVAPNNTSKTCSKCGHLNNYFSFEYRKKNKFPHFKCEKCNFKEDADYNAALNISNPKLKSTKEEP

SEQ ID NO: 38 - protein, 726 aa, synthetic construct
SEVEFSHEYWMRHALTLAKRARDEREVPVGAVLVLNNRVIGVGWNRAIGLHDPTAHAEIMALRQGGLVTQNYRLIDATLYVTFEPCVMCAGAMIHSRIGRVVFGVRNSKHGAAGSLVNVLNYPGMNHRVEITEGILADECAALLCDFYRMPRQVFNARKKAQSSIDPSGSSGGSSGSVTPGTSESATPESSGGGFGGSAKNTITKTLQLRIVRPYNSAEVEKIVADEKNNREKIALEKNKDKVKEACSKHLKVASYCTTQVERSACLFCKARKLDDKFYQKLRGQFPDAVFWQELGEIFRQLQKQAAEIYNQSLIELYYEIFIKGKGFANASSVEHYLSDVCYTRAAELFKNAAIASGLRGKVKSNFRLKELKNMKSGLPTTKSDNFPIPLVKQKGGQYTGFEISSHNDDFIIKIPFGRWQVKKEIDKYRPWEKFDFEQVRKSPKPISLLLSTQRRKRNKGWSKDEGTEAEIRKVMNGDYQTSYIEVKRGSKTGEKSAWMLNLSIDVPKIDKGVDPSIIGGIDVGVKSPLVCAINNAFSRYSISDNDLFRFNKKMFARRRILLKKNRHRRAGHGAKNKLKPITILTEKCKRFRKKLIERWACEIADFFIKNKVGTVQMENLESMKRKEDSYFNIRLRGFWPYAEMQNKIEFKLKQYGIEIRKVAPNNTSKTCSKCGHLNNYFNFEYRKMNKFPHFKCEKCNFKENADYNAALNISNPMLKSTKEEP

SEQ ID NO: 39 - protein, 726 aa, synthetic construct
SEVEFSHEYWMRHALTLAKRARDEREVPVGAVLVLNNRVIGEGWNRAIGLHDPTAHAEIMALRQGGLVMQNYRLIDATLYVTFEPCVMCAGAMIHSRIGRVVFGVRNNKHGAAGSLVNVLNYPGMNHRVEITEGILADECAALLCDFYRMPRQVFNARKKAQSSINPGGSSGSSSGSETPSTSESATPKSSGGSSGGSAKNTITKTLKLRIVRPYNSAEVEKIVADEKNNREKIALEKNKDKVKEACSEHLKVAAYCTTQVERNACLFCRARKLDDKFYQKLRGQFPDAVFWQEIGEIFRQLQKQAAEIYNQSLIELYYEIFIKGKGFANASSVEHYLSDVCYTRAAELFKNAAIASGLRGKVKSNFRLKELKNMKSGLPTTKSDNFPIPLVKQKGGQYTGFEISSHNDDFIIKIPFGRWQVKEEIDKYRPWEKFDFEQVRKSPKPISLLLSTQRRKRNKGWSKDEGTEAEIRKVMNGDYQTSYIEVKRGSKIGEKSAWMLNLSIDVPKIDKGVDPSIIGGIDVGVKSPLVCAINNALSRYSISDNDLFHFNRKMFARRRILLRKNRHKRAGHGARNKLKPITVLTEKSERFREKLIERWACEIANFFIKNKVGAVQMENLESMKRREDSYFNIRLRGFWPYAEMQSKIEFKLKQYGIKIRKVAPNNTSKTCSRCGHLNNYFNFEFRKKNKFPRFKCEKCNFKEDADYNAALNISNPKLKSTKEEP

SEQ ID NO: 40 - protein, 726 aa, synthetic construct
SEVEFSHEYWMRHALTLAKRARDEREVPVGAVLVLNNRVIGEGWNRAIGLHDPTAHAEIMALRQGGLVMQNYRLSDATLYVTFEPCVMCAGAMIHSRIGRVVFGVRNSKRGAAGSLMNVLNYPGMNHCVEITEGILVDECAALLCDFYRMPRQVLSAQKKAQSSVSSGGSSGGSSGSETPGASGSATPKSSVGSSAGPTKNTITKTLKLRIVRPYNSAEVEKIVADEKNNRERIALEKNKDKVKEACSKHLKMASYCTTQVERNACLFCKARKLDDKFYQKLRGQFPDAVFWQELGGIFRQLQKQAAEIYNQSLIELYYEIFIKGKGITNASRVEHYLSDVCYTRAAELFKNAAIASGLRSKVRSNFRLKELKNMKSGLPTTKSDNFPIPLVKQKGGQYTGFEISSHNDDFIIKIPFGRWHVKKEIDKYRPWEKFDFEQVRKGPKPISLLLSTQRRKRNKGWSKDEGTEAEIRKVMNGDYQTSYIEVKRGSKIGEKSAWMLNLSIDVPKIDKGVDPSIIGGIDVGVKSPLVCAINNAFSRYSISDNDLFRFNKKMFARRRILLRKNRHKRAGHGAKNKLKPISILTGKSERFRKKLIERWACEIADFFIKNKVGTVQMENLESMKRKEDSYFNIRLRGFWPYAEMQNKIEFKLKQYGIEIRKVAPNNTSKTCSKCGHLNNYFNFEYRKKNKFPHFKCEKCNFKEDADYNAALNISNPKLKSTKEEP

SEQ ID NO: 41 - protein, 726 aa, synthetic construct
SEVEFSHEYWMRHALSLAKRARDEREVPVGAVLVLNNRIIGEGWNRAIGLHDPTAHAEIMALRQGGLVMQNYRLTDATLYVTFEPCVMCAGAMVHSRIGRVVFGVRNSKRGAAGSLMNVLNYPGMNHRVEITEGVLADECAALLCDFYRMPRQVLNAQKKAQSSINSGGSSGGGSGGETPGTSESATQESSGGSSGGSAKNTITKTLKLRIVRPYNSAEVEKIVADEKNNREKIALEKNKDKVKEACSKHLKVAAYCTTQVERNACLFCKARKLDDKFYQKLRGQFPDAVFWQEISEIFRQLQKQAAVIYNQGLIELYYEIFIKGKGIANASRVEHYLSNVCYTRAAELFKNAAIASGLRNKIKSNFRLKELRNMKSGLPTTKSDNFPIPLVRQKGGQYTGFEISNHDGDFIIKIPFGRWQVKEEIDKYRPWEKFDFEQVRKSPKPISLLLSTQRRKKNKGWSKDEGTEAEIRRVMNGDYQTSYIEVKRGSKIGEKSAWMLNLSIDVPTIDKGVDPSIIGGIDVGVKSPLVCAINNSSSRYSICDNDLFRFNKKMFARRRILLKKNRHKRAGHGTKNKLKPITILTEKSGRFRKKLIERWACEIADFFIKNKVGTVQMENLESMKRKEDSYFNIRLRGFWPYAEMQNKIELKLKQYGIKIRKVAPNNTSKTCSRCGHLNDYFNFEYRKKNKFPHFKCEKCNLKEDADYNAALNISNPKLKSTKEEP

SEQ ID NO: 42 - protein, 726 aa, synthetic construct
SEVEFSHEYWMRHALTLAKRARDEREVPVGAVLVLNNRVIGEGWNRAIGLHDPTAHAEIMALRQGGLVMQNYRLTDATLYVTFEPCVMCAGAMIHSRIGRVVFGVRNSKRGAAGSLMNVLNYPGMNHCVEITEGILVDECAALLCDFYRMPRQVLNAQKKAQSSISSGGPTGGSSGSGTPGASGSVTPKSSGGSSAGSTKDTITKTLKLRIVRPYNSAEVEKIVADEKDNREEIALEKNKGKVKEACSKHLKVATYCTTQVERNACLFCKARKLDDKFYQKLRGQFPDAVFWQEIGEIFRQLQKQAAEIYNQSLIELYYEIFIKGKGFANASSVEHYLSDVCYTRAAELFKNAAIASGLRGKVKSNFRLKELKNMKSGLPTTKSDNFPIPLVKQKGGQYTGFEISSHNDDFIIKIPFGRWQVKKEIDKYRPWEKFDFEQVRKSPKPISLLLSTQRRKRNKGWSKDEGTEAEIKKVMNGDYQTSYIEVKRGSKIGEKSAWMLNLSIDVPKIDKGVDPSIIGGIDVGVRSPLVCAINNAFSRYSISDNDLFRFNKKMFARRRILLKKNRHKRAGHGAKNKLKPITIMTEKSKRFRKKLIERWACEIADFFIKNKVGTVQMENLESMKRREDSYFNIRLRGFWPYAEMQNKIEFKLKQYGIVVRKVAPNNTSKTCSKCGHLNNYFDFEYRKKNKFPHFKCEKCNFKEDADYNAALNISNPKLKSTKGEP

SEQ ID NO: 43 - protein, 726 aa, synthetic construct
SEVEFSHEYWMRHALTLAKRARDEREVPVGAVLVLNNRVIGEGWNRAIGLHDPTAHAEIMALRQGGLVMQNYRLTDATLYVTFEPCVMCAGAMIHSRIGRVVFGVRNSKHGAAGSLVNVLNHPGMNHRVEITEGILADECAALLCDFYRMPRQVFNAQKKAQSSISSGGSSGGSSGSKTPGTSESAAPESSGGSSGGSAKNTITKTLKLRIVRPYNSAEVEKIVADEKNNREKIALEKNKDKVKEACSKHLKVAAYCTTQVERNACLFCKARKLDDKFYQKLRGQFPDAVFWQEIGEIFRQLQKQAAEIYNQSLIELYYEILIKGKGIANASRVEHYLSDVCYTRAAELFKNAAIASGLRGKVKSNFRLKELKNMRSGLPTTKSDNFPIPLVKQKGGQYAGFEISSHNDDFIIKIPFGRWQVKKEIDKYRPWEKFDFEQVRKNPKPISLLLSTQRRKRNKGWSKDEGTEAEIRKVMNGDYQTSYIEVKRGSKIGEKSAWMLNLSIDVPKIDKGVDPSIIGGIDVGVKSPLVCAINNAFSRYSISDNDLFRFNKKVFARRRILLKKNRHKRAGRGAKNKLKPISILTEKSKRFRKKLIERWACEIADFFIKNKVGTVQMENLESMKRKEDSYFNIRLRGFWPYAEMQNKIEFKLKQYGIEIRKVAPNNTSKTCSKCGHLNNYFNFEYRKRNKFPHFKCEKCNFKENADYNAALNISNPKLKSTKEEP

SEQ ID NO: 44 - protein, 726 aa, synthetic construct
SEVEFSHEYWMRHALTLAKRARDEREVPVGAVLVLNNRVIGEGWNRAIGLHDPTAHAEIMALRQGGLVMQNYRLVDATLYVTFEPCVMCAGAMIHSRIGRVVFGVRNSKRGAAGSLMNVLNYPGMNHCVEITEGILVDECAALLCDFYRMPRQVLSAQKKAQSSVSSGDSSGGSSGSETPGASGSVTPKSSVGSSAGSTKNTITKTLKLRIVRPYNSAEVEKIVADEKNNREKIALEKNRDKVKEACSKHLKVAAYCTTQVERNACLFCKARKLDDKFYQKLRGQFPDAVFWQEIGEIFRQLQKQAAEIYNQSLIELYYEIFIKGKGFANASSVEHYLSDVCYTRAAELFKNAAIASGLRGKVKSNFRLKELKNMKSGLPTTKSDNFPIPLVKQKGGQYTGFEISSHNDDFIIKIPFGRWQVKKEIDKYRPWEKFDFEQVRKSPKPISLLLSTQRRKRNKGWSKDEGTEAEIRKVMNGDYQTSYIEVKRGSKIGEKGAWMLNLSIDVPKIDKGVDPSIIGGIDVGVKSPLVCAINNAFSRYSISDNDLFRFNKKMFARRRILLKKNRHKRAGHGAKNKLKPISILTGKSERFRKKLIERWACEIADFFIKNKVGTVQMENLESMKRKEDSYFNIRLRGFWPYAEMQNKIEFKLKQYGIEVRKVAPNNTSKTCSKCGHLNNYFNFEYRKKNKFPHFKCEKCNFKENADYNAALNISNPELKSTKEKP

SEQ ID NO: 45 - protein, 726 aa, synthetic construct
SEVEFSHEYWMRHALTLAKRARDEREVPVGAILVLNNRVIGVGWNRAVGLHDPTAHAEIMALRQGGLVMQNYRLVEATLYVTFEPCVMCAGAMIHSRIGRVVFGVRNSKRGAAGSLMNVLNYPGMNHCVEITEGILVDECAALLCDFYRMPRQVLNAQKKAQSSISSGGSSGGSSCSETPGASESVTPKSSGGSSAGSTKNTITKTLKLRIVRPYNSAEVEKIVADEKNSREKIALEKNKDKVKEACSEHLKVAAYCTTQVERNACLFCKARKLDDRFYQKLRGQFPDAVFWQEIGEIFRQLQKQAAEIYNQSLIELYYEIFIKGKGITNASRVEHYLSDVCYTRAAELFKNAAIASGLRSKVRSNFRLKELKNMKSGLPTTKSDNFPIPLVRQKGGQYTGFEISSHNDDFIIKIPFGRWQVKKEIDKYRPWERFDFEQVRKSPKPISLLLSTQRRKRNKGWSKDEGTEAEIRKVMNGDYQISYIEVKRGSKIGEKSAWMLNLSIDVPKIDKGVDPSIIGGIDVGVKSPLVCAINNALSRYSISDNDLFHFNKKMFARRRILLRKNRHKRAGHGAKNKLKPITIMTEKSKRFRKKLIERWACEIADFFIKNKVGTVQMENLESMKRKEDSYFNIRLRGFWPYAEMQSKIEFKLKQYGIVVRKVAPNNTSKTCSKCGHLNNYFNFEYRKKNRFPHFKCEKCNFKEDADYNAALNISNPKLKSTKGEP

SEQ ID NO: 46 - protein, 726 aa, synthetic construct
SEVEFSHEYWMRHALTLAKRARDEREVPVGAVLVLNNRVIGEGWNRAIGLHDPTAHAEIMALRQGGLVMQNYRLIDATLYVTFEPCVMCAGAMIHSRIGRVVFGVRNGKRGAAGSLMNVLNYPGMNHCVEITEGILVDECAALLCDFYRMPRQVLNAQKKAQSSISSGGSSGGSNGSETRGASESATPKSSGGSSGGSAKNTITKTLKLRIVRPYNSAEVEKIVADEKNNRERIALEKNKDKVKEACSKHLKVAAYCTTQVERNACLFCKARRLDDKFYQKLRGQFPDAVFWQELGEIFRQLQKQAAEIYNQSLIELYYEIFIKGKGFANASSVEHYLSDVCYTRAAELFKNAAIASGLRGKVKSNFRLKELKNMKSGLPTTKSDNFPIPLVRQKGGQYTGFEISNHNGDFIIKIPFGRWQVKKEIDKYRPWEKFDFEQVRKSPKPISLLLSTQRRKRNKGWSKDEGTEAEIRKVMNGDYQTSYIEVKRGSKIGEKSAWMLNLSIDVPKIDKGVDPSIIGGIDVGVKSPLVCAINNAFSRYSISDNDLFHYNKKMFARRRILLKKNRHKRAGHGAKNKLKPISILTEKSKRFRKKLIERWACEIADFFIKNKVGTVQMENLESMKRKEDSYFNIRLRGFWPYAEMQNKIEFKLKQYGIEIRKVAPNNTSKTCSKCGHLNNYFNFEYRKMNKFPHFKCEKCNFKENADYNAALNISNPKLKSTKGEP

SEQ ID NO: 47 - protein, 726 aa, synthetic construct
SEVEFSHEYWMRHALTLAKRARDEREVPVGAVLVLNNRVIGEGWNRAIGLHDPTAHAEIMALRQGGLAMQNYRLVDATLYVTFEPCVLCAGAMVHSRIGRVVFGVRNSKRGAAGSLMNVLNHPGMNHRVEITGGILADECAALLCDFYRMPRQVFNAQKKARSNINSGGSSGGSSDSETPGASESVTPKSSGGSSGGSAKNTITKTLKLRIVRPYNSAEVEKIVADEKNNREKIALEKNKGKVKEACSKHLEVAAYCTTQVERNACLFCKARKLDDKFYQKLRGQFPDAVFWQELGEIFRQLQKQAAEIYNQSLIELYYEIFIKGKGFANASSVEHYLSDVCYTRAAELFKNAAIASGLRGKVKSNFRLKELKNMKSGLPTTKSDNFPVPLVKQKGGQYTGFEISSHNDDFIIKIPFGRWQVKKEIDKYRPWEKFDFEQVRKSPKPISLLLSTQRRKRNKGWSKDEGTEAEIRKVMNGDYQTSYIEVKRGSKIGEKSAWMLNLSIDVPKIDKGVDPSIIGGIDVGVKSPLVCAISNAFSRYSISDNDLFHFNKKMFARRRILLKKSKHKRAGHGAKNKLKPITILTEKSRRFRKKLIERWACEIADFFIRNKVGTVQMENLESMKRKEDSYFNIRLRGFWPYAEMQNRIEFKLKQHGIEIRKVAPNNTSKTCSKCGHLNNYFNFEYRKKNKFPHFKCEKCNFKENADYNAALNISNPKLKSTKEEP

SEQ ID NO: 48 - protein, 726 aa, synthetic construct
SEVEFSHEYWMRHALTLAKRARDEREVPVGAVLVLNNRVIGEGWNRATGLHDPTAHAEIMALRQGGLVMQNYRLFDATLYVTFEPCVMCAGAMIHSRIGRVVFGVRNSKRGAAGSLMNVLNYPGMNHCVEITEGILVDECAALLCDFYRMPRQVLSAQKKAQSSVSSGGSSGGSSGSETPGASGSVTPKSSVGSSAGSTKNTITKTLKLRIVRPYNSAEVEKIVADEKNNREKIALEKNKGKVKEACSKHLKVASYCTTQVERNACPFCKARKLDDKFYQKLRGQFPDAVFWQELGGILRQLQKQAAEIYNQSLIELYYEIFIKGRGFANASSVEHYLSDVCYTRAAELFKNAAIASGLRGKVKSNFRLKELRNMKSGLPTTKSDNFPIPLVKQKGGQYTGFEISSHNDDFIIKIPFGRWQMKKEIDKYRPWEKFDFGQVRKSPKPISLLLSTQRRKRNKGWSKDEGTEAEIRKVMNGDYQTSYIEVKRGSKIGEKSAWMLNLSIDVPKIDKGVDPSIIGGIDVGVKSPLVCAINNAFSRYSISDNDLFHFNKKMFARRRILLKKNRHKRAGHGAKNKLKPISILTEKSKRFRKKLIERWACEIADFFIKNKVGTVQMENLESMKRKEDSYFNIRLRGFWPYAEMQSKIEFKLKQYGIEIRKVAPNNTSKTCSKCGHLNNYFNFEYRRKNKFPHFKCEKCNFKEDADYNAALNISNPKLKSTKEEP

SEQ ID NO: 49 - protein, 726 aa, synthetic construct
SEVEFSHEYWMRHALTLAKRARDEREVPVGAVLVLNNRVIGEGWNRAIGLHDPTAHAEIMALRRGGLVMQNYRLTDATLYVTFEPCVMCAGAMIHSRIGRVVFGVRNSKRGAAGSLMNVLNYPGMNHCVEITEGILVDECAALLCDFYRMPRQVLSAQKKAQSSISPGGSSGGSSGSETPGASESVTPKSSGGSSGGSAKNTITKTLKLRIVRPYNSAEVEKIVADEKNNREKIALEKNKGKVKEACSEHLKVAAYCTTQVERNACLFCKARKLDDRFYQKLRGQFPDAVFWQELGEILRQLQKQAAEIYNQSLIELYYEIFIKGKGFANASSVEHYLSDVCYTRAAELFKNAAIASGLRGKVKSNFRLKELRNMKSGLPTTKSDNFPIPLVRQKGGQYTGFEISSHNDDFIIKIPFGRWQVRKEIDKYRPWEKFDFEQVRKSPKPISLLLSTQRRKRNKGWSKDEGTEAEIRRVMNGDYQTSYIEVKRGSKIGEKSAWMLNLSIDVPKIDKGVDPSIIGGIDVGVKSPLVCAINNAFSRYSISDNDLFRFNKKMFARRRILLKKNRHKRAGHGAKNKLKPISILTRKSERFRKKLIERWACEIADFFIKNKVGTVQMENLESMKRREDNYFNIRLRGFWPYAEMQNKIEFKLKQYGIVVRKVAPNNTSKTCSKCGHLNNYFNFEYRKKNKFPHFKCEKCNFKEDADYNAALNISNPKLKSTKGEP

SEQ ID NO: 50 - protein, 726 aa, synthetic construct
SEVEFSHEYWMRHALTLAKRARGEREVPVGAVLVLNNRVIGEGWNRAIGLHDPTAHAEIMALRQGGLVMQNYRLTDATLYVTFEPCVMCAGAMIHSRIGRVVFGVRNSKRGAAGSLMNVLNYPGMNHCVEITEGILMDECAALLCDFYRMPRQVLNAQKKAQSSISSGGPSGGSSCSETPGASESVTPTSSGGSSTGSTKNTITKTLKLRIVRPYNSAEVEKIVADEKNSREKIALEKNKDKVKEACSKHLKMASYCTTQVERNACLFCKARKLDDKFYQKLRGQFPDAVFWQELGGIFRQLQKQAAEIYNQSLIELYYEIFIKGKGITNASRVEHYLSDVCYTRAAELFKNAAIASGLRSKVRSNFRLKELKNMKSGLPTTKSDNFPIPLVKQKGGQYTGFEISSHNDDFIIKIPFGRWQAKKEIDKYRPWEKFDFEQVRKSPKPISLLLSTRRRKRNKGWSKDEGTEAEIRKVMNGDYQTSYIEVKRGSKIGEKSAWMLNLSIDVPRIDKGVDPGIIGGIDVGVKSPLVCAINNAFGRYSISDNDLFHFNKKMFARRRILLKKNRHKRAGHGAKNKLKPITILTEKSKRFRKKLIERWACEIADFFIKNKVGTVQMENLESMKRKEDSYFNIRLRGFWPYAEMQDKIEFKLKQYGIEIRKVAPNNTSKTCSRCGHLNDYFNFEYRRKNKFPHFKCEKCNFKEDADYNAALNISNPKLKSTKGEP

SEQ ID NO: 51 - protein, 726 aa, synthetic construct
SEDEFSHEYWMRHALTLAKRARDEREVPVGAVLVLNNRVIGEGWNRAIGLHDPTAHAEIMALRQGGLVMQNYRLTEATLYVTFEPCVMCAGAMIHSRIGRVVFGVRNSKRGAAGSLMNVLNYPGMNHCVEITEGILVDECAALLCDFYRMPRQVLNAQKKAQSSISSGGSSGGSSGSETPGASESATPKSSVGSSAGSTKNTITKTLKLRIVRPYNSAEVEKIVADEKNNRERIALEKNKDKVKEACSKHLKVAAYCTTLVERNACLFCKARRLDDKFYQKLRGQFPDAVFWQEIGEIFRQLQKQAAEIYNQSLVELYYEILIKGKGIANASSVEHYLSDVCYTRAAKLFKNAAIASGLRNKIKSNFRLKELRNMKSGLPTTKSDNFPIPLVRQKGGQYTGFEISNHNDDFIIKIPFGRWQVKEEIDKYRPWEKFDFEQVRRNPKPISLLLSTQRRKRNKGWSKDEGTEAEIRKVMNGDYRTSYIEVKRGSKIGEKSAWMLNLSIDVPKIDKGVDPSITGGIDVGVKSPLVCAINNAFSRYSISDNDLFRFNKKVFARRRILLKKNRHKRAGHGARNKLKPITVLTEKSERFRKKLIERWACEIANFFIKNKVGTVQMENLESMKRREDSYFNIRLRGFWPYAEMQSKIEFKLKQYGIKIRKVAPNNTSKTCSRCGHLNNYFSFEYRKKNKFPHFKCEKCNFKEDADYNAALNISNPKLKSTKEEP

SEQ ID NO: 52 - protein, 726 aa, synthetic construct
SEVEFSHEYWMRHALTLAKRARDEREVPVGAVLVLNNRVIGEGWNRAIGLHDPTAHAEIMALRQGGLVMQNYRLTDATLYVTFEPCVMCAGAMIHSRIGRVVFGVRNSKRGAAGSLMNVLNYPGMNHCVEITEGILVDECAALLCDFYRMPRQVLNAQKKAQSSISSGGSSGGSSGNETPGASESATPKSSGGSSAGSTKDTITKTLKLRIVRPYNSAEVEKVVADEKNNREKIAIEKYKDMVKEACSKHLKVASYCTTQVERNACLFCKARKLDDKFYQKLRGQFPDAVFWQELGGIFRQLQKQAAEIYNQSLIELYYEIFIKGKGITNASRVEHYLSDVCYTRAAELFKNAAIASGLRNKIKSNFRLKELRNMKSGLPTTKSDNFPIPLVRQKGGQYTGFEISNHDGDFIIKIPFGRWQVKKEINKHRPWEKFDFEQVRKSPKPISLLLSTQRRKRNKGWSKDEGTEAEIRKVMNGDYQTSYIEVKRGSKIGEKSAWMLNLSIDVPKIDKGVDPGIIGGIDVGVKSPLVCAINNASSRYSISDNDLFHFNKKMFARRRILLKKNRHKRAGHGAKNKLKPITIMTEKSKRFRKKLIERWACEIADFFIKNKVGTVQMENLESMKRKEDSYFNIRLRGFWPYAEMQNKIEFKLKQYGIEIRKVAPNNTSKTCSKCGHLNYYFNFEYRKKNKFPHFKCEKCNFKENADYNAALNISSPKLKSTREEP

SEQ ID NO: 53 - protein, 726 aa, synthetic construct
SEVEFSHEYWMRHALTLAKRARDEREVPVGAVLVLNNRVIGEGWNRAIGLHDPTAHAEIMALRQGGLVTQNYRLIDATLYVTFEPCVMCAGAMIHSRIGRVVFGVRNNKHGAAGSLVNVLNYPGMNHRVEITEGILADECAALLCDFYRMPRQVFNARKRAQSSINPGGSSGGSGGSETPGTSESATPESSGGSPGSSAKNTITKTLKLRIVRPYNSAEVEKIVADEKNNREKIALEKNKDKVKEACSKHLKVAAYCTTQVERNACLFCKARRLDDKFYQKLRGQFPDAVFWQEIGEIFRQLQKQAAEIYNQSLVELYYEILIKGKGIANASSVEHYLSDVCYTRAAELFKNAAIASGLRNKIKSNFRLKELRNMRSGLPTTKSDNFPIPLVRQKGGQYTGFEISNHDGDFIIKIPFGRWQVKKEINKHRPWEKFDFEQVRKNPKPISLLLSTQRRKRNKGWSKDEGTEAEIRKVMNGDYQTSYIEVKRGSRTGEKSAWMLNLSIDVPKIDKGVDPSIIGGIDVGVKSPLVCAINNAFSRYSISDNDLFHFNKKMFARRRILLKRNRHKRAGHGTKNKLKPITILTEKSGRFRKKLIERWACEIANFFIKNKVGTVQMENLESMKRKEDSYFNIRLRGFWPYAEMQNKIEFKLKQYGIKIRKVAPNNTSKTCSKCGHLNNYFNFEYRKKNKFPHFKCEKCNFKENADYNAALNISNPKLKSTKEEP

SEQ ID NO: 54 - protein, 726 aa, synthetic construct
SEVEFSHEYWMRHALTLAKRARDEREVPVGAVLVLNNRVIGGGWNRAIGLHDPTAHAEIMALRQGGLVMQNCRLVDATLYVTFEPCVMCAGAMIHSRIGRVVFGVRNSKRGAAGSLMNVLNYPGMNHRVEITEGILVDECAALLCDFYRMPRQVFNAQKRAQSTINTGGSSGGSSGSETPGTSESPTPESSGGNSGGSAKNTITKTLTLRIVRPYNSAEVEKIVADEKNNREKIALEKNKDKVKEACSTHLKVATYCTTQVERNACLFCKARKLDDKFYQKLRGQFPDAVFWQEIGEIFRQLQKQAAEIYNQSLIELYYEIFIKGKGFANASSVEHYLSDVCYTRAAELFKNAAIASGLRGKVKSNFRLKELKNMKSGLPTTKSDNFPIPLVKQKGGQYTGFEISSHNDDFIIKIPFGRWQVKKEIDKYRPWEKFDFAQVRKSPKPISLLLSTQRRRRNRGWSKDEGTEAEIKKVMNGDYQISYIEVKRGSKIGEKSAWMLSLSVDVPKIDKGVDPSIIGGIDVGVKSPLVCAINNALSRYSISDNDLFHYNKKMFARRRILLKKNRHKRAGHGTKNKLKPITILTEKSGRFRKKLIERWACEIANFFIKNKVGTVQMENLESMKRKEDSYFNIRLRGFWPYAEMQNKIEFKLKQYGIKIRKVAPNNTSKTCSKCGHLNNYFSFEYRKKNKFPHFKCEKCNFKEDADYNAALNISNPKLKSTKEEP

SEQ ID NO: 55 - protein, 726 aa, synthetic construct
SEVEFSHEYWMRHALALAKRARDEREVPVGAVLVLNNRVIGEGWNRAIGLHDPTAHAEIMALRQGGLVMQNYRLTDATLYVTFEPCVMCAGAMIHSRIGRVVFGVRNSKRGAAGSLMNVLNYPGMNHCVEITEGILVDECAALLCDFYRMPRQVLNAQKKAQSSISSGGSSGGSSGSETPGASGSVTPKSSGGSSGGSAKNTITKALKLRIVRPYNSAEVEKIVADEKNNRERIALEKNKGKVKEACSKHLKVAAYCTTQVERNACLFCKARKLDDKFYQKLRGQFPDAVFWQEIGEIFRQLQKQAAEIYNQSLIELYYEIFIKGKGIANASSVEHYLSDVCYTRAAELFKNAAIASGLRNKIKSNFRLKELRNMKSGLPTTKSDNFPIPLVRQKGGQYTGFEISNHNGDFIIKIPFGRWQVKKEIRKHRPWEKFDFEQVRKSPKPISLLLSTQRRKRNKGWGKDEGTEAEIRKVMNGDYQTSYIEVKRGSKIGEKSAWMLSLSIDVPKIDKGVDPSIIGGVDVGVKSPLVCAINNAFSRYSISDNDLFRFNKRMFARRRILLKKNRHKRAGHGAKNKLKPITIMTEKSKRFRKKLIERWACEIADFFIKNKVGTVQMENLESMKRKEDSYFNIRLRGFWPYAEMQNKIEFKLKQYGIEIRKVAPNNTSKTCSKCGHLNYYFNFEYRKKNKFPHFKCEKCNFKEDADYNAALNISNPKLKSTKEEP

SEQ ID NO: 56 - protein, 726 aa, synthetic construct
SEVEFSHEYWMRHALTLAKRARDEREVPVGAVLVLNNRVIGEGWNRAIGLHDPTAHAEIMALRQGGLVLQNYRLVDATLYVTFEPCVLCAGAMVHSRIGRVVFGARNSKRGAAGSLMNILNYPGMNHRVEITEGILADECAALLCDFYRMPRQVFNAQKKAQSSINSGGSSGGSSGSETPSTSESATPESSGGSSGGSAKNTITKTLQLRIVRPYNSAEVEKIVTDEKNNREKIALEKNKDKVKEACSKHLKMASYCTTQVERNACLFCKARELDDKFYQKLRGQFPDAVFWQELGGIFRQLQKQAAEIYNQSLIELYYEIFIKGKGITNASRVEHYLSDVCYTRAAELFKNAAIASGLRSKVRSNFRLKELKNMRSGLPTTKSDNFPIPLVKQKGGQYTGFEISSHNSDFIIKIPFGRWQVKEEIDKFRPWEKFDFEQVRKSPKPISLLLSTQRRKKNKGWSKDEGTEAEIRRVMNGDYQTSYIEVKRGSKIGEKSAWMLNLSIDVPKIDKGVDPSIIGGIDVGVKSPLVCAINNSSSRYSICDNDLFHFNKKMFARRRILLKKNRHKRAGHGAKNKLKPITILTEKSKRFRKKLIERWVCEVADFFIKNKVGTVQMENLESMKRKEDSYFNIRLRGFWPYAEMQNRIELKLKQYGIEIRRVAPNNTSRTCSKCGHLNNYFNFEYRKKNKFPHFKCEKCNFREDADYNAALNISNPKLKSTKEEP

SEQ ID NO: 57 - protein, 726 aa, synthetic construct
SEVEFSHEYWMRHALTLAKRARDKHEVPVGAVLVLDNRVIGEGWNRATGQNDPTAHAEIMALRQGGLVMQNHRLIDATLYVTFEPCVMCAGAMIHSRIGRVVIGVRNSKRGAAGSLMNVLNHPGMNHRVEITEGILADECAALLCDFYRMPRQVLNAQEKAQSSINSGGSSGGSSGSETPGTSESATPGSSGGSSGGSAKNTITKTLKLRIVRPYNSAEVEKIVADEKNSREKTALERNKDKVKEACSKHLKMAAYCTTQVERNACLFCKARKLDDKFYQKLRGQFPDAVFWQEVGEIFRQLQKQAAEIYNQSLIELYYEIFIKGKGFANASSVEHYLSDVCYTRAAGLFKNAAIASGLRGKVKSNFRLKELKNMKSGLPTTKSDNFPIPLVKQKGGQYTGFEISSHNDDFIIKIPFGRWQVKKEIDKYRPWEKFDFEQVRKSPKPISLLLSTRRRKRNKGWSKDEGTEAEIRKVMNGDYQTSYIEVKRGSKIGEKSAWMLNLSIDVPKIDKGVDPSIIGGIDVGVKSPLVCAINNAFSRYSISDNDLFRFNKKMFARRRILLKKNRHKRAGHGAKNKLRPISILTGKSERFRKKLIERWACEIADFFIKNKVGTVQMENLESMKRKEDSYFNIRLRGFWPYAEMQNKIELKLKQYGIKIRKVAPNNTSKTCSKCGHLNDYFNFEYRKKNKFPHFKCEKCNFKEDADYNAALNISNPKLKSTREEP

SEQ ID NO: 58 - protein, 726 aa, synthetic construct
SEVEFSHEYWMRHALTLAKRARDEREVPVGAILVLNNRVIGVGWNRAIGLHDPTAHAEVMALRQGGLVTQNYRLIDATLYVTFEPCVMCAGAMIHSRIGRVVFGVRNSKHGAAGSLVNVLNYPGMNHRVEITEGILADECAALLCDFYRMPRQVFNARKKAQSSINPGGSSGGSSDSEAPGTSENATPGSSGGSSGGSAKNTITKTLKLRIVRPYNSAEVEKIVADEKNNREKIALEKNKDKVKEACSEHLKVAAYCTTQVERNACLFCKARKLDDKFYQKLRGQFPDAVFWQELGGIFRQLQKQAAEIYNQSLIELYYEIFIKGKGITNASRVEHYLSDVCYTRAAELFKNAAIASGLRSKVRSNFRLKELKNMKSGLPTTKSDNFPIPLVKQKGGQYTGFEISSHNSDFIIKIPFGRWQAKEEIDKYRPWEKFDFEQVRKSPKPISLLLSTQRRKKNKGWSKDEGTEAEIRRVMNGDYQTSYIEVKRGSKVGEKSTWMLNLSIDVPKIDKGVDPSIIGGIDVGVKSPLVCAINNSSSRYSICDNDLFRFNKKMFARRRILLKKNRHKRAGHGAKNKLKPITIMTEKSKRFRKKLIERWACEIADFFIKNKVGTVQMENLESMKRKEDSYFNIRLRGFWPYAEMQNKIEFKLKQYGIEIRKVAPNNTSKTCSKCGHLNNYFNFEYRKMNKFPHFKCEKCNFKENADYNAALNISNPKLKSIKEEP

SEQ ID NO: 59 - protein, 726 aa, synthetic construct
SEVEFSHEYWMRHALTLAKRARDEREVPVGAVLVLNNRVIGEGWNRAVGLHDPTAHAEIMALRQGGLVMQNYRLTDATLYVTFEPCVMCAGAMIHSRIGRVVFGVRNSKRGAAGSLMNVLNYPGMNHCVEITEGILMDECAALLCDFYRMPRQVLIAQKKAQSSISSGGSSGGSSCSETPGASESVTPKSSGGSSAGSTRNTITKTLKLRIVRPYNSAEVEKIVADEKNSREKIALEKNKDKVKEACSEHLKVAAYCTTQVERNACLFCKARKLDDRFYQKLRGQFPDAVFWQETGEIFRQLQRQAAEIYNQSLIELYYEIFIKGKGFANASSVEHYLSDVCYTRAAELFKNAAIASGLRGKVKSNFRLKELKNMKSGLPTTKSDNFPIPLVKQKGGQYTGFEISSHNDDFIIKIPFGRWQVKKEIDKYRPWEKFDFEQVRKSPKPISLLLSTQRRKRNKGWSKDEGTEAEIRKVMNGDYQTSYIEVKRGSKIGEKSAWMLNLSIDVPKIDKGVDPGIIGGIDVGVKSPLVCAINNALSRYSISDNDLFHFNKKMFARRRILLRKNRHKRAGHGAKNKLKPITIMTEKSKRFRKKLIERWACEIADFFIKNKVGTVQMENLESMKRKEDSYFNIRLRGFWPYAEMQNKIEFKLKQYGIVVRKVAPNNTSKTCSKCGHLNNYFNFEYRKKNKFPHFKCEKCNFKEDADYNAALNISNPKLKSTKGEP

SEQ ID NO: 60 - protein, 726 aa, synthetic construct
SEVEFSHEYWMRHALTLAKRARDEREVPVGAVLVLNNRVIGEGWNRAIGLHDPTAHAEIMALRQGGLVLQNYRLADATLYVTFEPCVLCAGAMVHSRIGRVVFGARNSKRGAAGSLMNILNYPGMNHRVEITEGILADECAALLCDFYRMPRQVFSVRRKAQSSISPGGSSGGSSGSETPGTGKSPTPESPGGSSGGSAKNTITKTLKLRIVRPYNSAEVEKIVADEKNNREKIALERNKDKVKEACSEHLKVAAYCTTQVERNACLFCKARKLDDKFYQKLRGQFPDAVFWQETGEIFRQLQKQAAEIYNQSLIELYYEIFIKGKGFANASSVEHYLSDVCYTRAAELFKNAAIASGLRGKVKSNFRLKELKNMKSGLPTTKSDNFPIPLVKQKGGQYTGFEISSHNDDFIIKIPFGRWQVKKEINKYRPWEKFDFEQVRKSPKPISLLLSTQRRKRNKGWSKDEGTEAEIRKVMSGDYQTSYIEVKRGSKIGEKSAWMLNLSIDVPKIDKGVDPSIIGGIDVGVKSPLVCAINNAFSRYSISDNDLFRFNKKMFARRRILLGKNRHKRAGHGVKNKLKPITILTEKSGRFRKKLIERWACEIADFFVKNKVGTVQMENLESMKRKEDSYFNIRLRGFWPYAEMQNKIEFKLKQYGIKIRKVAPNNTSKTCSKCGHLNNYFNFEYRKKNKFPHFKCEKCNFKEDADYNAALNISNPKQKSTKEEP

SEQ ID NO: 61 - protein, 726 aa, synthetic construct
SEVEFSHEYWMRRALTLAKRARDEREVPVGAVLVLNNRVIGVGWNRAVGLHDPTAHAEIMALRQGGLVMQNYRLIEATLYVTFEPCIMCAGAMIHSRIGRVVFGVRNSKRGAAGSLMNVLNYPGMNHRVEITEGILADECAALLCDYYRMPRQVFNARKKAQSSTNSGGSSDGGSGSETPGTSESATPESSGGSSGGSAKNTITKTLTLRIVRPYNSAEVEKIVADEKNNREKIALEKNKDKVKEACSEHLKVATYCTTQVERNACPFCKARKLDDKFYQKLRGQFPDAVFWQELGEIFRQLQKQAAEIYNQSLIELYYEIFIKGKGFANASSVEHYLSDVCYTRAAELFKNAAIASGLRGKVKSNFRLKELRNMKSGLPTTKSDNFPIPLVRQKGGQYTGFEISSRNDDFIIKIPFGRWQVKKEIDKYRPWEKFDFEQVRKSPKPISLLLSTQRRKRNRGWGKDEGTEAEIKRVMNGDYQTSYIEVKRGSKIGEKSAWMLNLSIDVPKIDKGVDPSIIGGIDVGVKSPLVCAINNAFSRYSISDNDLFHFNKKMFARRRILLKKNRHKRAGHGAKNKLKPISILTEKSKRFRKKLIERWACEIADFFIKNKVGTVQMENLESMKRKEDSYFNIRLRGFWPYAEMQNKIEFKLKQYGIEIRKVAPNNTSKTCSKCGHLNSYFNFEYRKKNKFPHFKCEKCNFKEDADYNAALNISNPKLKSTKEGP

SEQ ID NO: 62 - protein, 726 aa, synthetic construct
SEVEFSHEYWMRHALTLAKRARDEREVPVGAVLVLNNRVIGEGWNRAIGLHDPTAHAEIMALRQGGLVMQNYRLIEATLYVTFEPCIMCAGAMIHSRIGRVVFGVRNSKRGAAGSLMNVLNYPGMNHRVEITEGILADECAALLCDYYRMPRQVFNARKKAQSSINSGGSSDGGSGSETPGTSESATPESSGGSSGGSAKNTITKTLKLRIVRPYNSAEVEKIVADEKNNREKIALEKNKDKVKEACSEHLKVAAYCTTQVERNACLFCKARKLDDKFYQKLRGQFPDAVFWQEIGEIFRQLQKQAAEIYNQSLIELYYEIFIKGRGFANASSVEHYLSDVCYTRAAELFKNAAIASGLRGKVKSNFRLKELKNMKSGLPTTKSDNFPIPLVKQKGGQYTGFEISSHNDDFIIKIPFGRWQVKKEINKFRPWEKFDFEQVRKSPKPISLLLSTQRRKRNKGWSKDEGTEAEIRKVMNGDYQTSYIEVKRGSKTGEKSTWMLNLSIDVPKIDKGVDPSIIGGIDVGVKSPLVCAINNAFSRYSISDNDLFRFNKKMFARRRILLKKNRHKRAGHGAKNKLKPISILTEKSKRFRKKLIERWACEIADFFIKNKVGIVQMENLESMKRKEDSYFNIRLRGFWPYAEMQNKIEFKLKQYGIEIRKVAPNNTSKTCSKCGHLNNYFNFEYRKKNKFPHFKCEKCNFKENADYNAALNISNPMLKSTKEEP

SEQ ID NO: 63 - protein, 726 aa, synthetic construct
SEVEFSHEYWMRHALTLAKRARDEHEVPVGAVLVLNNRAIGEGWNRAIGLHDPTAHAEIMALRQGGLVMQNYRLTDATLYVTFEPCVMCAGAMIHSRIGRVVFGVRNSKHGAAGSLVNVLNYPGMNHRVEITEGILADECAALLCDFYRMPRQVFNARKKAQSSISSGGSSGGSSGSVTPGASGSVTPKSSGGSSAGSTKDTITKTLKLRIVRPYNSAEVEKIVADEKNNREKIALEKNKDMVKEACSKHLKVASYCTTQVERNACPFCKARKLDDKFYQKLRGQFPDAVFWQELGEILRQLQKQAAEIYNQSLVELYYEIFIKGKGITNASRVEHYLSDVCYTRAAELFKNAAIASGLRSKVRSNFRLKELKNMKSGLPTTKSDNFPIPLVKQKGGQYTGFEISSHNDDFIIKIPFGRWQVRKEIDKYRPWEKFDFEQVRRSPKPISLLLSTQRRKRNKGWSKDEGTEAEIKRVMNGDYQTSYIEVKRGSKIGEKSAWMLSLSIDVPKIDKGVDPSIIGGIDVGVKSPLVCAINNALSRYSISDNDLFHFNKKMFARRRILLRKNGHKRAGHGAKNKLKPITILTEKSVRFRKKLIERWACEIADFFVKNKVGTVQMENLESMKRKEDSYFNIRLRGFWPYAEMQNKIEFKLKQYGIEIRKVAPNNTSKTCSKCGHLNSYFNFEYRKKNKFPHFKCEKCNFKENADYNAALNISNPKLKSTKEEP

SEQ ID NO: 64 - protein, 726 aa, synthetic construct
SEVEFSHEYWMRHALTLAKRARDEREVPVGAVLVLNNRVIGEGWNRTTGLHDPTAHAEIMALRQGGLVMRNYRLTDATLYVTFEPCVMCAGAMIHSRIGRVVFGVRNSKRGAAGSLMNVLNYPGMNHRVEITEGILVDECAALLCDFYRMPRRVLNAQKKAQSSISSGGSSGGSSGSETPGASESVTPKSSVGSSASSTKNTITKTLKLRIVRPYNSAEVEKIVADEKDNREKIALEKNKDKVKEACSKHLKVAAYCTTQVERNACLFCKARKLDDKFYQKLRGQFPDAVFWQEVSEIFRQLQKQAAEIYNQSLIELYYEIFIKGKGFANASSVEHYLSDVCYTRAAELFKNAAIASGLRGKVKSNFRLKELKNMKSGLPTTKSDNFPIPLVKQKGGQYTGFEISSHNDDFIIKIPFGRWQVKKEIDKYRPWEKFDFEQVRKSPKPISLLLSTQRRKRNKGWSKDEGTEAEIRKVMNGDYQTSYVEVKRGSKIGEKSAWMLSLSIDVPKIDRGVDPSIIGGIDVGVKSPLVCAINNAFSRYSISDNDLFHFNKKVFARRRILLKKNRHRRVGHGAKNKLKPITILTEKSKRFRKKLIERWACEIADFFIKNKVGTVQMENLESMKRKEDSYFNIRLRGFWPYAEMQNKIEFKLKQYGIEIRKVAPNNTSKTCSKCGHLNNYFNFEYRKKNKFPHFKCEKCNFKENADYNAALNISNPKLKSTKEKP

SEQ ID NO: 65 - protein, 726 aa, synthetic construct
SEVEFSHEYWMRHALTLAKRARDEREVPVGAVLVLNNRVIGEGWNRAIGLHDPTAHAEVMALRQGGLVMQNYRLTDATLYVTFEPCVMCAGAMIHSRIGRVVFGVRNSKRGAAGSLMNVLNYPGMNHCVEITEGILVDECAALLCDFYRMPRQVLNAQKKAQSSISPGGSSGGSSGSETPGASGSVTPKSSGGSSAGSTRDTITKTLKLRIVRPYNSAEVEKIVADEKNNREKIALEKNKDKVKEACSEHLKVAAYCTTQVERSACLFCKARKLDDKFYQKLRGQFPDAVFWQEIGEIFRQLQKQAAEIYNQSLIELYYEIFIKGKGFANASSVEHYLSDVCYTRAAELFKNAAIASGLRGKVKSNFRLKELKNMRSGLPTTKSDNFPIPLVKQKGGQYTGFEISSHNDDFIIKIPFGRWRVKKEIDKYRPWEKFDFEQVRKSPKPISLLLSTQRRKRSKGWSKDEGTEAEIRKVMNGDYQTSYIEVKRGSKIGEKSAWMLSLSIDVPKIDKGVDPSIIGGIDVGVKSPLVCAINNALSRYSISDNDLFHFNKKMFARRRILLRKNRHKRAGHGVRNKLKPITVLTEKSERFRKKLIERWACEIANFFIKNKVGTVQMENLESMKRREDSYFNIRLRGFWPYAEMQSKIEFKLKQYGIEIRKVAPNNTSKTCSKCGHLNNYFNFEFRKKNKFPHFKCEKCNFKEDADYNAALNISNPKLKSTKEEP

SEQ ID NO: 66 - protein, 726 aa, synthetic construct
SEVEFSHEYWMRHALTLAKRARDEREVPVGAILVLNNRVIGEGWNRAIGLHDPTAHAEIMALRQGGLVMQNYRLTDATLYVTFEPCVMCAGAMIHSRIGRVVFGVRNSKRGAAGSLMNVLNYPGMNHCVEITEGILVDECAALLCDFYRMPRQVLNAQKKAQSSISSGGSSGGSSGSKTPCASESATPKSSGGSSGGSAKNTITKTLQLRIVRPYNSAEVEKIVTDEKNNREKIALEKNKDKVKEACSKHLKMASYCTTQVERNACLFCKARKLDDKFYQKLRGQFPDAVFWQELGGIFRQLQKQAAEIYNQSLIELYYEIFIKGKGITNASRVEHYLSDVCYTRAAELFKNAAIASGLRSKVRSNFRLKELKNMKSGLPTTKSDNFPIPLVKQKGGQYTGFEICSHNDDFIIKIPFGRWQVKKEIDKYRPWEKYDFEQVRKSPKPISLLLSTQRRKRNKGWSKDEGTEAEIRKVMNGDYQTSYIEVKRGSKTGEKSAWMLNLSIDVPKIDKGVDPSIIGGIDVGVKSPLVCAINNAFSRYSISDNDLFRFNKKMFARRRILLRKNRHKRAGHGAKNKLKPISILTGKSERFRKKLIERWACEIADFFIKNRVGTVQMENLESMKRKEDSYFNIRLRGFWPYAEMQNKIEFKLKQYGIEIRKVAPNNTSKTCSKCGHLNNYFNFEYRKKNKFPHFKCEKCNFKENADYNAALNISNPKLKSTKEEP

SEQ ID NO: 67 - protein, 726 aa, synthetic construct
SEVEFSHEYWMRHALTLAKRARDEREVPVGAVLVLNNRVIGEGWNRAIGLHDPTAHAEIMALRQGGLVMQNYRLIDATLYVTFEPCVMCAGAMIHSRIGRVVFGVRNNKHGAAGSLVNVLNYPGMNHRVEITEGILADECAALLCDFYRMPRQVFNARKKAQSSINPGGSSGGSSGSETPGTSESATPESSGGSSGSPAKNTITKTLKLRIVRPYNSAEVEKIVADEKNNREKIALEKNKDKVKEACSKHLKVAAYCTTQVERNACLFCKARRLDDKFYQKLRGQFPDAVFWQEIGEIFRQLQKQAAEIYNQSLIELYYEIFIKGKGITNASRVEHYLSDVCYTRAAELFKNAAIASGLRGKVKSNFRLKELKNMKSGLPTTKSDNFPIPLVKQKGGQYTGFEISSHNDDFIIKIPFGRWQVKEEIDKYRPWEKFDFEQVRKNPKPISLLLSTLRRKRNKGWSKDEGTEAEIRKVMNGDYQTSYIEVKRGSKIGEKSAWMLNLSIDVPKIDKGADPSVIGGIDVGVKSPLVCAINNAFSRYSISDNDLFRFNKKMFARRRILLGKNRHKRAGHGVKNKLKPITILTEKSGRFRKKLIERWACEIADFFVKNKVGTVQMENLESMKRKEDSYFNIRLRGFWPYAEMQNKIEFKLKQYGIKVRKVAPNNTSKTCSKCGHLNNYFSFEYRKKNKFPHFKCEKCNFKENADYNAALNISNPKLKSTKEEP

SEQ ID NO: 68 - protein, 726 aa, synthetic construct
SEVEFSHEYWMRHALTLAKRARDEREVPVGAVLVLNNRVIGEGWNRAIGLHDPTAHAEIMALRQGGLVMQNYRLTDATLYVTFEPCVMCAGAMIHSRIGRVVFGVRNSKRGAAGSLMNVLNYPGMNHCVEITEGILVDECAALLCDFYRMPRQVLNAQKKAQSSISPGGSSGGSSGSETPGASGSVTPKSSGGSSAGSTKDTITKTLKLRIVRPYNSAEVEKIVADEKNNREKIALEKNKGKVKEACSKHLKVATYCTTQVERNACLFCKARRLDDKFYQKLRDQFPDAVFWQEIGEIFRQLQKQAAEIYNQSLVELYYEIFIKGKGIANASSVEHYLSDVCYTRAAELFKNAAIASGLRNKIKSNFRLKELRNMKSGLPTTKSDNFPIPLVRQKGGQYTGFEISNHNGDFIIKVPFGRWQVKKEINKYRPWEKFDFEQVRKSPKPISLLLSTQRRKKNKGWSKDEGTEAEIRRVMNGDYQTSYIEVKRGSKIGEKSAWMLNLSIDVPKIDKGVDPSIIGGIDVGVKSPLVCAINNAFSRYSISDNDLFRFNKKMFARRRILLGKNRHKRAGHGVKNKLKPITILTEKSGRFRKKLIERWACEIADFFVKNKVGTVQMENLESMKRKEDSYFNIRLRGFWPYAEMQNKIEFKLKQYGIKVRKVAPNNTSKTCSKCGHLNNYFNFEYRRKNKFPHFKCEKCNFKEDADYNAALNISNPKLKSTKEEP

SEQ ID NO: 69 - protein, 726 aa, synthetic construct
SEVEFSHEYWMRHALTLAKRARDEREVPVGAVLVLNNRVIGEGWNRAIGLHDPTAHAEIMALRQGGLVMQNYRLTDATLYVTFEPCVMCAGAMIHSRIGRVVFGVRNSKRGAAGSLMNVLNYPGMNHCVEITEGILMDECAALLCDFYRMPRQVLSAQKRAQSSISSGGPSGGSSCSETPGASESVTPKSSGGSSTGSTKNTITKTLKLRIVRPYNSAEVEKIVADEKNNREKIALEKNKDKVKEACSKHLKVASYCTTQVERNACPFCKARKLDDKFYQKLRGQFPDAVFWQELGEILRQLQKQAAEIYNQSLIELYYEIFIKGKGFANASSVEHYLSDVCYTRAAELFKNAAIASGLRGKVKSNFRPKELKNMKSGLPTTKSDNFPIPLVKQKGGQYTGFEISSHNDDFIIKIPFGRWQVKEEIDKYRPWEKFDFEQVRKNPKPISLLLSTQRRKRNKGWSKDEGTEAEIRKVMNGDYQTSYIEVKRGSKIGEKSAWMLNLSIDVPKIDKGVDPSIIGGIDVGVKSPLVCAINNAFSRYCISDNDLFRFNKKVFARRRILLKKNKHKRAGHGTKNKLKPITILTEKSGRFRKKLIERWACEIADFFIKNKVGTVQMENLESMKRKEDSYFNIRLRGFWPYAEMQNKIELKLKQYGIKIRKVAPNNTSKTCSKCGHLNDYFNFEYRKKNKFPHFKCEKCNFKEDADYNAALNISNPKLKSTREEP

SEQ ID NO: 70 - protein, 726 aa, synthetic construct
SEVEFSHEYWMRHALTLAKRARDEREVPVGAVLVLNNRVIGEGWNRAIGLHDPTAHAEIMALRQGGLVMQNYRLTDATLYVTFEPCVMCAGAMIHSRIGRVVFGVRNSKRGAAGSLMNVLNYPGMNHRVEITEGILADECAALLCDYYRMPRQVFNARKKAQSSINSGGSSGGSSGSETPGTSESATPESSGGGSSGSAKNTITKTLQLRIVRPYNSAEVEKIVADEKNNREKIALEKNKDKVKEACSKHLKVAAYCTTQVERNACLFCRARKLDDKFYQKLRGQFPDAVFWQEIGEIFRQLQKQAAEIYNQSLIELYYEIFIKGKGIANASSVGHYLSDVCYTRAAELFKNAAIASGLRGKVKSNFRLKELKNMRSGLPTTKSDNFPIPLVKQKGGQYAGFEISSHNDDFIIKIPFGRWQVKKEIDKYRPWEKFNFEQVRKSPKPISLLLSTQRRKRNKGWSKDEGTEAEIRKVMNGDYQTSYIEVKRGSKTGEKSAWMLNLSIDVPKIDKGVDPSIIGGIDVGVKSPLVCAINNAFSRYSISDNDLFRFNKKMFARRRILLKKNRHKRAGHGAKNKLKPITILTEKSKRFRKKLIERWACEIANFFIKNKVGTVQMENLESMKRREDSYFNIRLRGFWPYAEMQSKIEFKLKQYGIEVRKVAPNNTSKTCSKCGHLNNYFNFEFRKKNKFPHFKCEKCNFKEDADYNAALNISNPKLKSTKEVP

SEQ ID NO: 71 - protein, 726 aa, synthetic construct
SEVEFSHEYWMRHALTLAKRARDKHEVPVGAVLVLDNRVIGEGWNRATGQNDPTAHAEIMALRQGGLVMQNHRLIDATLYVTFEPCVMCAGAMIHSRIGRVVIGVRNSKRGAAGSLMNVLNHPGMNHRVEITEGILADECAALLCDFYRMPRQVFNAQEKAQSSINSGGSSGGSSGSETPGTSESATPGSSGGSSGGSAKNTITKTLKLRIVRPYNSAEVEKIVADEKNSREKIALEKNKDKVKEACSKHLRVAAYCTTQVERNACLFCKARKLDDKFYRKLRGQFPDAVFWQELGEIFRQLQKQAAEIYNQSLIELYYEIFVKGKGIANTSRMEHYLSDVCYTRAAKLFKNAAIASGLRGKIKSNFRLKELKSMKSGLPTTKSDNFPIPLVKQKGGQYTGFEISSHNDDFIIKIPFGRWQVKKEIDKYRPWEKFDFEQVRKSPKPISLLLSTQRRKRNKGWSKDEGTEAEIRKVMNGDYQTSYIEVRRGSKIGEKSAWMLSLSIDVPKIDKGVDPGIIGGIDVGVKSPLVCAINSASSRYSISDNDLFHFNKKMFARRRILLKKNGHKRAGHGAKNKLKPITIMTEKSKRFRKKLIERWACEIADFFIKNKVGTVQMENLESMRRKEDSYFNIRLRGFWPYAEMQNKIEFKLKQYGIEIRKVAPNNTSKTCSKCGHLNNYFNFEYRKKNKFPHFKCEKCNFKVNADYNAALNISNPKLKSTKEEP

SEQ ID NO: 72 - protein, 726 aa, synthetic construct
SEVEFSHEYWMRHALTLAKRARDEREVPVGAVLVLNNRVIGEGWNRAIGLHDPTAHAEIMALRQGGLVLQNYRLVDATLYVTFEPCVLCAGAMVHSRIGRVVFGARNSKRGAAGSLMNILNYPGMNHRVEITEGILADECAALLCDFYRMPRQVFNARKKAQSSINPGGSSGGSSGSETPGTSESTTPEGSGSSSGGSAKNTITKTLKLRIVRPYNSAEVEKIVADEKNNREKIALEKNKDKVREACNKHLKVASYCTTQVERNACPFCKARKLDDKFYQKLRGQFPDAVFWQELGEILRQLQKQAAEIYNQSLVELYYEILIKGKGIANASSVEHYLSDVCYTRAAELFKNAAIASGLRNKIKSNFRLKELRNMKSGLPTTKSDNFPIPLVRQKGGQYTGFEISNHDGDFIIKIPFGRWQVKKEINKHRPWEKFDFEQVRKSPKPISLLLSTQRRKRNKGWSKDEGTEAEIRKVMNGDYQTSYIEVKRGSKIGEKSAWMLNLSIDVPKIDKGVDPSIIGGIDVGVKSPLVCAINNALSRYSISDNDLFHFNKKMFARRRILLRKNRHKRAGHGTKNKLKPITIMTEKSKRFRKKLIERWACEIADFFIKNKVGTVQMENLESMKRKEDSYFNIRLRGFWPYAEMQSKIEFKLKQYGIVVRKVVPNNTSKTCSKCGHLNNYFNFEYRKKNKFPHFKCEKCNFKEDADYNAALNISNPKLKSTKGEP

SEQ ID NO: 73 - protein, 726 aa, synthetic construct
SEVEFSHEYWMRHALTLAKRARDEREVPVGAILVLNNRVIGEGWNRAIGLHDPTAHAEIMALRQGGLVMQNYRLIDATLYVTFEPCVMCAGAMIHSRIGRVVFGVRNNKHGAAGSLVNVLNYPGMNHRVEITEGILADECAALLCDFYRMPRQVFNARKKAQSSINPGGSSGGSSGSETPGTSESATPESSGGSSGSSAKNTITKTLKLRIVRPYNSAEVEKIVADEKNNREKIALEKNEGKVKEACSKHLEMAAYCTTQVERNACLFCKARKLDDKFYQKLGGQFPDAVFWQELGEIFRQLQKQAAEIYNQSLIELYYKIFIKGKGFANASSVEHYLSDVCYTRAAELFKNAAIASGLRGKVKSNFRLKELKNMKSGLPTTKSDNFPVPLVKQKGGQYTGFEISNHNGDFIIKIPFGRWQVKEEINKYRPWEKFDFEQVRKSPKPISLLLSTQRRKRNKGWSKDEGTEAEIRKVMNGDYQTSYIEVKRGGKIGEKSAWMLSLSIDVPKIDRGVDPSIVGGIDVGVKSPLVCAINNALGRFSISDNDLFHFNKKMFARRRILLRKNRHKRAGHGAKNKLKPISILTEKSKRFRKKLIERWACEIADFFIKNKVGTVQMEDLESMKRRGDSYFNIRLRGFWPYAEMQNKIEFKLKQYGIETRKVAPNNTSKTCSKCGHLNNYFNFEYRKRNKFPHFKCEKCNFKENADYNAALNISNPKLKSTKEKP

SEQ ID NO: 74 - protein, 726 aa, synthetic construct
SEVEFSHEYWMRHALTLAKRARDEREVPVGAVLVLNNRVIGEGWNRAIGLHDPTAHAEIMALRQGGLVMQNYRLIDATLYVTFEPCVMCAGAMIHSRIGRVVFGVRNNKHGAAGSLVNVLNYPGMNHRVEITEGILADECAALLCDFYRMPRQVFSAQKKAQSSINPGSSSGGSSGSKTPGTSESATPESSGGGSGGSAQNTITKTLKLRIVRPYNSAVVEKIVADEKNNREKIALERNKDKVKEACSRHLKVAAYCTTQVERNACLFCKARKLDDKFYQKLRGQFPDAVFWQELGGIFRQLQKQAAEIYNQSLIELYYEIFIKGKGITNASRVEHYLSDVCYTRAAELFKNAAIASGLRSKVRSNFRLKELKNMKSGLPTTKSDNFPIPLVKQKGGQYTGFEISSHNDDFIIKIPFGRWQVKKEIDKYRPWEKFDFEQVRKSPKPISLLLSTQRRKRNKGWSKDEGTEAEIKKVMNGDYQTSYIEVKRGSKIGEKSAWMLNLSIDVPKIDKGVDPSIIGGIDVGVKSPLVCAINNAFSRYSISDNDLFHFNKKMFARRRILLKKNRHKRAGHGAKNKLRPLTILTGKSKRFRKKLIERWACEIADFFVKNKVGTVQMENLESMKRKEDSYFNIRLRGFWPYAEMQNKIEFKLKQYGIEVRKVAPNNTSKTCSKCGHLNNYFNFEYRKKNKFPHFKCEKCNFKENADYNAALNISNPKLKSTKEEP

SEQ ID NO: 75 - protein, 726 aa, synthetic construct
SEVEFSHEYWMRHALTLAKRARDEREVPVGAVLVLNNRVIGEGWNRAIGLHDPTAHAEIMALRQGGLVMQNYRLTDATLYVTFEPCVMCAGAMIHSRIGRVVFGVRNSKRGAAGSLMNVLNYPGMNHCVEITEGILMDECAALLCDFYRMPRQVLSAQKKAQSSISSGGPSGGSSCSETPGASESVTPKSSGGSSGGSAKNTFTKTLKLRIVRPYNSAEVEKIVADEKNNREKIALEKNKDKVKEACSEHLKVAAYCTTQVERNACLFCKARKLDDKFYQKLRGQFPDAVFWQEIGEIFRQLQKQAAEIYNQSLIELYYEIFIKGKGFANASSVEHYLSDVCYTRAAELFKNAAIASGLRGKVKSNFRLKELKNMRSGLPTTKSDNFPIPLVKQKGGQYAGFEISNHNSDFIIKIPFGRWQVKKEIDKYRPWEKFDFEQVRKSPKPISLLLSTRRRKKNKGWSKDEGTEAEIRKVMNGDYQTSYIEVKRGSKIGEKSAWMLNLSIDVPKIDKGVDPSIIGGIDVGVKSPLVCAINNAFSRYSISDNDLFRFNKKMFARRRILLKKNRHKRAGHGAKNKLKPISILTGKSERFRKKLIERWACEIADFFIKNKVGTVQMENLESMKRKEDSYFNIRLRGFWPYAEMQNKIEFKLKQYGIEIRKVAPNNTSKTCSKCGHLNNYFNFEYRKKNKFPHFRCEKCNFKENADYNAALNISNPKLKSTKEEP

SEQ ID NO: 76 - protein, 726 aa, synthetic construct
SEVEFSHEYWMRHALTLAKRARDEREVPVGAVLVLNNRVIGEGWNRAIGLHDPTAHAEIMALRQGGLVMQNYRLTDATLYVTFEPCVMCAGAMIHSRIGRVVFGVRNSKRGAAGSLMNVLNYPGMNHRVEITEGILVDECAALLCDFYRMPCQVLNAQKKAQSSISSGGSSGGSSGSDTLGASESVTPKSSVGSSASSTKNTITKTLKLRIVRPYNSAEVEKIVADEKDNREKIALEKNKDKVKEACSKHLKVAAYCTTQVERNACLFCKARKLDDKFYQKLRGQFPDAVFWQEIGEIFRQLQKQAAETYNQSLVELYYEILIKGKGIANASSVEHYLSDVCYTRAAELFKNAAIASGLRNKIKSNFRLKELRSMKSGLPTTKSDNFPIPLVRQKGGQYTGFEISSHNDDFIIKIPFGRWQVKKEIDKYRPWEKFDFEQVRKSPKPISLLLSTQRRKRNKGWSKDEGTEAEIRKVMNGDYQTSYIEVKRGSKAGEKSAWMLNLSIDVPKIDRGVDPSIIGGIDVGVKSPLVCAINNAFSRYSISDNDLFRFNKKMFARRRILLKKNRHKRAGHGAKNKLKPITILTEKSKRFRKKLIERWACEIADFFIKNKVGTVQMENLESMKRKEDSYFNIRLRGFWPYAEMQNKIEFKLKQYGIEIRKVAPNNTSKTCSKCGHLNNYFNFEYRRKNKFPHFKCERCNFKEDADYNAALNISNPKLKSTKEEP

SEQ ID NO: 77 - protein, 726 aa, synthetic construct
SEVEFSHEYWMRHALTLAKRARDEREVPVGAVLVLNNRVIGEGWNRAIGLHDPTAHAEIMALRQGGLVMQNYRLIDATLYVTFEPCVMCAGAMIHSRIGRVVFGVRNNKHGAAGSLVNVLDYPGMNHRVEITEGILADECAALLCDFYRMPRQVFNAQKKAQSSVSFGGSSGGSSGSETPGASGSVTPKSSVGSSAGSTKNTITKTLKLRIVRPYNSAEVEKIVADEKNNREKVALEKNKDKVKEACSKHLKVAAYCTTQVERNACLFCKARKLDDKFYQKLRGQFPDAVFWQEIGEIFRQLQKQAAEIYNQSLIELYYEIFIKGKGFANASSVEHYLSDVCYTRAAELFKNAAIASGLRGKVKSNFRLKELKNMKSGLPTTKSDNFPIPLVKQKGGQYTGFEISSHNDDLIVKIPFGRWQVKKEIDRYRPWEKFDFEQVRKSPKPISLLLSTQRRKRNKGWSKDEGTEAEIRKVMNGDYQISYIEVKRGSKIGEKNAWMLNLSIDVPKIDKGVDPSIIGGIDVGVKSPLVCAINNAFSRYSISDNDLFRFNKKMFARRRILLKKNRHKRAGHGAKNKLKPISILTEKSKRFRKKLIERWACEIADFFIKNKVGTVQMENLESMKRKEDSYFNIRLRGFWPYAEMQNKIEFKLKQYGIEIRKVAPNNTSKTCSKCGHLNNYFNFEYRRKNKFPHFKCEKCNFKENADYNAALNISNPKLKSTKEEP

SEQ ID NO: 78 - protein, 726 aa, synthetic construct
SEVEFSHEYWMRHALTLAKRARDEREVPVGAVLVLNNRVIGEGWNRAIGLHDPTAHAEIMALRQGGLVMQNYRLVDATLYVTFEPCVLCAGAMVHSRIGRVVFGVRNSKRGAAGSLMNVLNYPGMNHRVEITEGILADECAALLCDFYRMPRRVFNAREKARSNINSGGSSGGSSSSETPGTSGSATPEGSGGSSGGSAKNTITKTLKLRIVRPYNSAEVEKIVADEKNNREKIALEKNKDKVKEACSKHLKVASYCTTQVERNACLFCKARKLDDKFYQKLRGQFPDAVFWQELGEIFRQLQKQAAEIYNQSLIELYYEIFIKGKGFANASSVEHYLSDVCYTRAAELFKNAAIASGLRGKVKGNFRLKELKNMKSGLPTTKSDNFPIPLVKQKGGQYTGFEISSHNDDFIIKIPFGRWQVKKEIDKYRPWEKFDFEQVRKSPKPISLLLSTQRRKRNKGWSKDEGTEAEIRKVMNGDYQTSYIEVKRGSRIGEKSAWMLSLSIDVPKIDRGVDPSIIGGIDVGVKSPLVCAINNALSRYSISDNDLFHFNKKMFARRRILLKKSKHKRAGHGAKNKLKPITTLTEKSRRFRKKLIERWACEIADFFIKNKVGTVQMENLESMKRREDSYFNIKLRGFWPYAEMQNKIEFKLKQYGIEIRKVAPNNTSKTCSKCGHLNNYFNFEYRKKNKFPHFKCEKCNFKENADYNAALNISNPKLKGTKEEP

SEQ ID NO: 79 - protein, 726 aa, synthetic construct
SEVEFSHEYWMRHALTLAKRARDEREVPVGAVLVLNNRVIGEGWNRAIGLHDPTAHAEIMALRQGGLVMQDYRLSDATLYVTFEPCVMCAGAMIHSRIGRVVFGVRNSKRGAAGSLMNVLNYPGMNHCVEITEGILVDECAALLCDFYRMPRQVLSAQKKAQSSISSGGSSGGSSGSETPGASGSVTPKSSVGSSAGSTKNTITKTLKLRIVRPYNSAVVEKIVADEKNNREKIALEKNKDKVKEACSKHLKVASYCTTQVERNACPFCKARKLDDKFYQKLRGQFPDAVFWQELGEILRQLQKQAAEIYNQSLIELYYEIFIKGRGFANASSVEHYLSDVCYTRAAELFKNAAIASGLRGKVKSNFRLKELKNMKSGLPTTKSDNFPIPLVKQKGGQYTGFEISSHNDDFIIKIPFGRWQVKKEIDKFRPWEKFDFEQVRKSPKPISLLLSTQRRKRNKGWSKDEGTEAEIRKVMNGDYQTSYIEVKRGSKIGEKSAWMLNLSIDVPKIDKGVDPSIIGGIDVGVKSPLICAINNAFSRYGISDNDLFRFNKKVFARRRILLKKNRHKRAGHGTKNKLKPITILTEKSGRFRKKLIERWACEIANFFIKNKVGTVQMENLESMKRKEDSYFNIRLRGFWPYAEMQNKIEFKLKQYGIVVRKVAPNNTSKTCSKCGHLNNYFNFEYRKKNKFPHFKCEKCNFKEDADYNAALNISNPKLKSTKEEP

SEQ ID NO: 80 - protein, 726 aa, synthetic construct
SEVEFSHEYWMRHALTLAKRARDGREVPVGAVLVLNNRVIGEGWNRTTGLHDPTAHAEIMALRQGGLVMQNHRLVDATLYVTFEPCVMCAGAMIHSRIGRVVFGVRNSKRGAAGSLMNVLNYPGMNHCVEITEGILVDECAALLCDFYRMPRQVLNAQKKAQSSISSGGSSGGSSGSETPGASESVTPKSSVGSSAGSTKNTITKTLKLRIVRPYNSAEVEKIVADEKNNREKIALEKNKDKVKEACSEHLKVAAYCTTQVERSACLFCKARKLDDKFYQKLRGQFPDAVFWQELGGIFRQLQKQAAEIYNQSLIELYYEIFIKGKGITNASRVEHYLSDVCYTRAAELFKNAAIASGLRSKVRSNFRLKELKNMKSGLPTTKSDNFPIPLVKQKGGQYTGFEISSHNSDFIIKIPFGRWQVKKEIGKYRPWEKYDFEQVRKSPKPISLLLSTQRRKRNKGWSKDEGTEAEIRKVMNGDYQTSYIEVKRGSKTGEKSAWMLNLSIDVPKIDKGVDPSIIGGIDVGVKSPLVCAINNAFSRYSISDNDLFRFNKKMFARRRILLGKNRHKRAGHGVKNKLKPITILTEKSGRFRKKLIERWACEIADFFVKNKVGTVQMENLESMKRKEDSYFNIRLRGFWPYAEMQNKIEFKLKQYGIEIRKVAPNNTSKTCSKCGHLNNYFNFEYRKKNKFPHFKCEKCNFKENADYNAALNISNPKLKSTKEEP

SEQ ID NO: 81 - protein, 726 aa, synthetic construct
SEVEFSHEYWMRHALTLAKRARDEREVPVGAILVLNNRVIGEGWNRAIGLHDPTAHAEIMALRQGGLVMQNYRLIDATLYVTFEPCVMCAGAMIHSRIGRVVFGVRNNKHGAAGSLVNVLNYPGMNHRVEITEGILADECAALLCDFYRMPRQVFNARKKAQSSINPGGSSGSSSGSETPGTSESATPESSGGSSGGSAKNTITKTLKLRIVRPYNSAEVEKIVADEKNNREKIALEKNKGKVKEACSKHLKVAAYCTTLVERNACLFCKARRLDDKFYQKLRGQFPDAVFWQEIGEIFRQLQKQAAEIYNQSLIELYYEIFIKGKGFANASSVEHYLSDVCYTRAAELFKNAAIASGLRGKVKSNFRLKELKNMKSGLPTTKSDNFPIPLVKQKGGQYTGFEISSHNDDFIIKIPFGRWQVKKEIDKYRPWEKFDFEQVRKSPKPISLLLSTQRRKRNKGWSKDEGTEAEIRKVMNGDYQTSYIEVKRGSKIGEKSAWMLSLSIDVPKIDKGVDPSIIGGIDVGVKSPLVCAINNALSRYSISDNDLFRFNKKMFARRRILLKKNRHKRAGHGAKNKLKPITIMTEKSKRFRKKLIERWACEIADFFIKNKVGTVQMENLESMKRKEDSYFNIRLRGFWPYAEMQNKIEFKLKQYGIEIRKVAPNNTSRTCSKCGHLNNYFNFEYRKKNKFPHFKCEKCNFREDADYNAALNISNPKLKSTKEEP

SEQ ID NO: 82 - protein, 726 aa, synthetic construct
SEVEFSHEYWMRHALMLAKRARDEREVPVGAVLVLNNRVIGVGWNRAVGLHDPTAHAEIMALRQGGLVMQNYRLIEATLYVTFEPCIMCAGAMIHSRIGRVVFGVRNGKRGAAGSLMNVLNYPGMNHRVEITEGILADECAALICDYYRMPRQVLNAQKKAQSSISSGGSSGGSSCSETPGASESVTPKSSGGSSGGSAKNTITKALKLRIVRPYNSAEVEKIVADEKNNREKIALEKNKDKVKEACSKHLKVAAYCTTQVERNACLFCKARKLDDKFYQKLRGQFPDAVFWQEIGEIFRQLQRQAAEIYNRSLIELYYEIFIKGKGFANASSVEHYLSDVCYTRAAELFKNAAIASGLRGKVKSNFRLKELKNMKSGLPTTKSDNFPIPLVKQKGGQYTGFEISSHNDDFIIKIPFGRWQVKEEIDKYRPWEKFDFEQVRKSPKPISLLLSTQRRKRNKGWSKDEGTEAEIRKVMNGDYQTSYIEVKRGSKTGEKSAWMLNLSIDVPRIDKGVDPSIIGGIDVGVKSPLVCAINNAFGRYSISDNDLFHFNKKMFARRRILLKKNRHKRAGHGAKNKLKPITILTEKSKRFRKKLIERWACEIADFFIKNKVGTVQMENLESMKRKEDSYFNIRLRGFWPYAEMQDKIEFKLKQYGIEIRKVAPNNTSKTCSRCGHLNDYFNFEYRRKNKFPHFKCEKCNFKENADYNAALNISNPKLKSTKEEP

SEQ ID NO: 83 - protein, 726 aa, synthetic construct
SEVEFSHEYWMRHALTLAKRARDEREVPVGAILVLNNRVIGVGWNRAIGLHDPTAHAEIMALRQGGLVTQNYRLTDATLYVTFEPCVMCAGAMIHSRIGRVVFGVRNSKRGAAGSLMNVLNYPGMNHCVEITEGILMDECAALLCDFYRMPRQVLNAQKKAQSSISSGGPSGSSSCSETPGASESVTPKSSGGSSTGSTKNTITKTLQLRIVRPYNSAEVEKIVTDEKNNREKIALEKNKDKVKEACSKHLKMASYCTTQVERNACLFCKARKLDDKFYQKLRGQFPDAVFWQELGGIFRQLQKQAAEIYNQSLIELYYEIFIKGKGITNASRVEHYLSDVCYTRAAELFKNAAIASGLRGKVKSNFRLKELKNMKSGLPTTKSDNFPIPLVKQKGGQYTGFEISSHNDDFIIKIPFGRWQAKEEIDKYRPWEKFDFEQVRKSPKPISLLLSTQRRKRNKGWSKDEGTEAEIRKVMNGDYQTSYIEVKRGSKIGEKSAWMLNLSIDVPKIDKGVDPSIIGGIDVGVKSPLVCAINNAFSRYSIGDNDLFHFNKKMFARRRILLKKNKHRRAGHGVKNKLKPISILTEKSKRFRKKLIERWACEIADFFIKNKVGTVQMENLESMKRKEDSYFNIRLRGFWPYAEMQNKIEFKLKQYGIEIRKVAPNNTSKICSKCGHLNNYFNFEYRRKNKFPHFKCEKCNFKENADYNAALNVSNPKLKSTKEEP

SEQ ID NO: 84 - protein, 726 aa, synthetic construct
SEVEFSHEYWMRHALTLAKRARDEREVPVGAVLVLNNRVIGEGWNRAIGLHDPTAHAEIMALRQGGLVMQNYRLTDATLYVTFEPCVMCAGAMIHSRIGRVVFGVRNSKRGAAGSLMNVLNYPGMNHCVEITEGILMDECAALLCDFYRMPRQVLNAQKKAQSSISSGGPSGSSSCSETPGASESVTPKSSGGSSTGSTKNTITKTLKLRIVRPYNSAEVEKIVADEKNSREKIALEKNKDKVKEACSEHLKVAAYCTTQVERNACLFCKARKLDDRFYQKLRGQFPDAVFWQEIGEIFRQLQKQAAEIYNQSLIELYYEIFIKGKGFAIASSVEHYLSCVCYTRAAELFKNAAIASGLRGKVKSNFRLKELKNMKSGLPTTKSDNFPIPLVKQKGGQYTGFEICSHNDDFIIKIPFGRWQVKKEIDKYRPWEKFDFEQVRKSPKPISLLLSTQRRKRNKGWSKDEGTEAEIRKVMNGDYQISYIEVKRGRKIGEKSAWMLNLSIDVPKIDKGVDPSIVGGIDVGVKSPLVCAINNALGRYSISDNDLFHFNKKMFARRRILLKKNGHKRAGHGARNKLKPITVLTEKSKRFRKKLIERWACEIANFFIKNRVGTVQMEDLESMKRKEDSYFNIRLRGFWPYAEMQNRIEFKLKQYGIEIRKVAPNNTSKTCSKCGHLNNYFNFEYRKKNKFPHFRCEKCNFKENADYNAALNICNPKLKGTKEEP

SEQ ID NO: 85 - protein, 726 aa, synthetic construct
SEVEFSHEYWMRHALTLAKRARDEREVPVGAVLVLNNRVIGEGWNRAIGLHDPTAHAEIMALRQGGLVMQNNRLTDATLYVTFEPCVMCAGAMVHSRIGRVVFGVRNSKRGAAGSLMNVLNYPGVNHCVEITEGILVDECAALLCDFYRMPRHVLNAQKRAQSSISSGGSSGGCSGSEMPGASESVTPKSSGGSSAGSTKNTITKTLKLRIVRPYNSAEVEKIVADEKNSREKIALERNKDKVKEACSEHLKVAPYCTTRVERNACPFCKARKLDDKFYQKLRGQFPDAVFWQELGEILRQLQKQAAEIYNQSLIELYYEIFIKGRGFANASSVEHFLSDVCYTRAAELFKNAAIASGLRGKVKSNFRLKELKNMKSGLPTTKSDNFPIPLVKQKGGQYTGFEISSHNDDFIIKIPFGRWQVKKEIDKYRPWEKFDFEQVRKSPKPISLLLSTQRRKRNKGWSKDEGTEAEIRKVMNGDYQTSYIEVKRGSKTGEKSTWMLNLSIDVPKIDKGVDPSIIGGIDVGVKSPLVCAINNAFSRYSISDNDLFRFNKKMFARRRILLKKNRHKRAGHGAKNKLKPISVLTEKSGRFRKKLIERWACEIADFFIKNKVGTVQMENLGSMKRKEDSYFNIRLRGFWPYAEMQNKIEFKLKQYGIEIRKVAPDNTSKTCSKCGHLNNYFNFEYRKKNKFPHFKCEKCNFKEDADYNAALNISNPKLKSTKEEP

SEQ ID NO: 86 - protein, 726 aa, synthetic construct
SEVEFSHEYWMRHALTLAKRARDEREVPVGAILVLNNRVIGEGWNRAIGLHDPTAHAEIMALRQGGLVMQNYRLIDATLYVTFEPCVMCAGAMIHSRIGRVVFGVRNSKHGAAGSLVNVLNYPGMNHRVEITEGILADECAALLCDFYHMPRQVFNARKRAQSSINSGGSSGGSSGSGTPGTSESATPKSSGGSSGGSAKNTITKALKLRIVRPYNSAEVEKIVADEKNNREKIALEKNKDKVKEACSKHLKVASYCTTQVERNACPFCKARKLDDKFYQKLRGQFPDAVFWQELGEILRQLQKQAAEIYNQSLIELYYEIFIKGRGFANAGSVEHYLSDVCYTRAAELFKNAAIASGLRGKVKSNFRLKELKNMKSGLPTTKSDNFPIPLVKQKGGQYTGFEISSHNDDFIIKIPFGRWQVKKEIDKYRPWEKFDFEQVRKSPKPISLLLSTQRRKRNKGWSKDEGTEAEIRKVMNGDYQTSYIEVKRGSKTGEKSAWMLNLSIDVPKIDKGVDPSIIGGIDVGVKSPLVCAINNAFSRYSISDNDLFRFNKKMFARRRILLKKSRHKRAGHGAKNKLKPITILTEKSRRFRKKLIERWACEIADFFIKNKVGTVQMENLESMKRKEDSYFNIRLRGFWPYAEMQNKIEFKLKQYGIVIRKVAPNNTSRTCSKCGHLNNYFNFEYRKKNKFPHFKCEKCNFKENADYNAALNISNPKLKSTKEEP

SEQ ID NO: 87 - protein, 726 aa, synthetic construct
SEVEFSHEYWMRHALTLAKRARDEREVPVGAVLVLNNRVIGEGWNRTTGLHDPTAHAEIMALRQGGLVMQNHRLIDATLYVTFEPCVMCAGAMIHSRIGRVVFGVRNSKRGAAGSLMNVLNYPGMNHRVEITEGILADECAALLCDFYRMPRRVFNAQKKAQSSINSSGSSGGSSGSETPGTSESATPESFGGSSGGSAKNTITKTLKLRIVRPYNSAEVEKIVADEKNSREKIALEKNKGKVKEACSEHLKVAAYCTTQVERSACPFCKARKLDDRFYQKLRGQFPDAVFWQELGGIFRQLQKQAAEIYNQSLIELYYEIFIKGKGITNASRVEHYLSDVCYTRAAELFKNAAIASGLRSKVRSNFRLKELKNMKSGLPTTKSDNFPIPLVKQKGGQYTGFEISSHNDDLIIKIPFGRWQVKKEIDKYRPWEKFDFEQVRKSPKPISLLLSTQRRKRNKGWSKDEGTEAEIRKVMNGDYQTSYIEVKRGSKIGEKSAWMLNLSIDVPKIDKGVDPSIIGGIDVGVKSPLVCAINNAFSRYSISDNDLFRFNKKMFARRRILLGKNRHKRAGHGVKNKLKPITILTEKSGRFRKKLIERWACEIADFFVKNKVGTVQMENLESMKRKEDSYFNIRLRGFWPYAEMQNKIEFKLKQYGIKVRKVAPNNTSKTCSKCGHLNNYFSFEYRKKNKFPHFKCEKCNFKENADYNAALNISNPKLKSTKEEP

SEQ ID NO: 88 - protein, 726 aa, synthetic construct
SEVEFSHEYWMRHALTLAKRARDEREVPVGAILVLNNRVIGEGWNRAIGLHDPTAHAEIMALRQGGLVMQNYRLIDATLYVTFEPCVMCAGAMIHSRIGRVVFGVRNSKHGAAGSLVNVLNYPGMNHRVEITEGILADECAALLCDFYRMPRQVFSARRKAQSSISPGGSSGGSSGGETPGSSKSLTPESPGGSSGGSAKNTITKTLKLRIVRPYNSAEVEKIVADEKNNREKIALEKNKDKVKEACGKHLKVAAYCTTQVERNACLFCKARKLDDKFYQKLRGQFPDAVFWQEIGEIFRQLQKQAAEIYNRSLIELYYEIFIKGKGFANASSVEHYLSDVCYTRAAELFKNAAIASGLRGKVKSNFRLKELKSMKSGLPTTKSDNFPIPLVKQKGGQYTGFEISSHNDDFIIKIPFGRWQVKKEIDKYRPWEKFDFEQVRKNPKPISLLLSTQRRKRNKGWSKDEGTEAEIRKVMNGDYQTSYIEVKRGSKIGEKSAWMLNLSIDVPKIDKGVDPSIIGGIDVGVKSPLVCAINNAFSRYSISDNDLFRFNKKVFARRRILLKKNRHKRAGHGTKNKLKPITILTEKSGRFRKKLIERWACEIANFFIKNKVGTVQMENLEGMKRKEDSYFNIRLRGFWPYAEMQNKIEFKLKQYGIKIRKVAPNNTSKTCSKCGHLNNYFSFEYRKKNKFPHFKCEKCNFKEDADYNAALNISNPKLKSTKEEP

SEQ ID NO: 89 - protein, 726 aa, synthetic construct
SEVEFSHEYWMRHALSLAKRARDEREVPVGAVLVLNNRIIGEGWNRAIGLHDPTAHAEIMALRQGGLVMQNYRLTDATLYVTFEPCVMCAGAMVHSRIGRVVFGVRNSKRGAAGSLMNVLNYPGANHCVEITEGILVDECAALLCDFYRMPRQVLNAQKKAQSSISSGGSSGGCSGSEMPGASESVTPKSSGGSSGGPAKNTITKTLKLRIVRPYNSAEVEKIVADEKNNREKIALEKNKGKVKEACSKHLEVAAYCTTQVERNACLFCKARKLDDKFYQKLRGQFPDAVFWQELGEIFRQLQKQAAEIYNQSLIELYYEIFIKGKGFANASSVEHYLSDVCYTRAAELFKNAAIASGLRGKVKSNFRLKELKNMKSGLPTTKSDNFPIPLVKQKGGQYTGFEISSHNDDFIIKIPFGRWQVKKEINKFRPWEKFDFEQVRKSPKPISLLLSTQRRKRNKGWSRDEGTEAEIRKVMNGDYQTSYIEVKRGSKIGEKSAWMLNLSIDVPKIDKGVNPSIIGGIDVGVKSPLVCAINNAFSRYSISDNDLFRFNKKMFARRRILLGKNRHKRAGHGVKNKLKPITILTEKSGRFRKKLIERWACEIADFFVKNKVGTVQMENLESMKRKEDSYFNIRLRGFWPYAEMQNKIEFKLKQYGIKVRKVAPNNTSKTCSKCGHLNNYFSFEYRKKNKFPHFKCERCNFKENADYNAALNISNPKLKSTKGEP

SEQ ID NO: 90 - protein, 726 aa, synthetic construct
SEVEFSHEYWMRHALTLAKRARDEREVPVGAVLVLNNRVIGEGWNRAIGLHDPTAHAEIMALRQGGLVLQNYRLVDATLYVTFEPCVLCAGAMVHSRIGRVVFGARNSKRGAAGSLMNILNYPGMNHRVEITEGILADECAALLCDFYRMPRQVFNAQKKAQSSINSGGSSGGSSGSETPSTSESATPESSGGSSGGSAKNTITKTLQLRIVRPYNSAEVEKIVTDEKNNREKIALEKNKDKVKEACSKHLKMASYCTTQVERNACLFCKARKLDDKFYQKLRGQFPDAVFWQELGGIFRQLQKQAAEIYNQSLIELYYEIFIKGKGFANASSVEHYLSDVCYTRAAELFKNAAIASGLRGKVKSNFRLKELKNMKSGLPTTKSNNFPIPLVKQKGGQYTGFEISSHNDDFIIKIPFGRWQVKKEIDKYRPWEKFDFEQVRKSPKPISLLLSTQRRKRNKGWSKDEGTEAEIRKVMNGDYQTSYIEVKRGSKTGEKSAWMLSLSIDVPKIDKGVDPSIIGGIDVGVKSPLVCAINNAFSRYSISDNDLFRFNKKMFARRRILLKKNRHKRAGHGAKNKLKPISILTRKSERFRRKLIERWACEIADFFIKNKVGTVQMENLESMKRKEDSYFNIRLRGFWPYAEMQNKIEFKLKQYGIEIRKVAPNNTSKTCSKCGHLNNYFNFEYRKKNKFPHFKCEKCNFKENADYNAALNISNPKLKSTKEEP

SEQ ID NO: 91 - protein, 726 aa, synthetic construct
SEVEFSHEYWMRHALTLAKRARDEREVPVGAVLVLNNRVIGEGWNRAIGLHDPTAHAEIMALRQGGLVMRNYRLTDATLYVTFEPCVMCAGAMIHSRIGRVVFGVRNSKRGAAGSLMNVLNYPGMNHCVEITEGILVDECAALLCDFYRMPRQVLNAQKKAQSSISPGGSSGGSSGSETPGASESVTPKSSGGSSGGSAKNTITKTLKLRIVRPYNSAEVEKIVADEKNNRERIALEKNKDKVREACSKHLKVASYCTTQVERNACLFCKARKLDDKFYQKLRGQFPDAVFWQELGEIFRQLQKQAAEIYNQSLIELYYEIFIKGKGFANASSVEHYLSDVCYTRAAELFKNAAIASGLRGKVKSNFRLKELKNMKSGLPTTKSDNFPIPLVKQKGGQYTGFEISSHNDDFIIKIPFGRWQAKKEIDKYRPWEKFDFEQVRKSPKPISLLLSTQRRKRNKGWSKDEGTEAEIRKVMNGDYQTSYIEVKRGSKIGEKSAWMLNLSIDVPKIDKGVDPSIIGGIDVGVKSPLVCAINNAFSRYSISDNDLFHFNKKVFARRRILLKKNRHKRAGHGVKNKLKSISILTEKSKRFRKKLIERWACEIADFFIKNKVGTVQMENLESMKRREDSYFNIRLRGFWPYAEMQNKIEFKLKQYGIEIRKVAPNNTSKTCSKCGHLNNYFNFEYRKKNKFPHFKCEKCNFKENADYNAALNISNPKLKSTKEEP

SEQ ID NO: 92 - protein, 726 aa, synthetic construct
SEVEFSHEYWMRHALTLAKRARDEREVPVGAVLVLNNRVIGEGWNRAIGLHDPTAHAEIMALRQGGLVMQNYRLTDATLYVTFEPCVMCAGAMIHSRIGRVVFGVRNSKRGAAGSLMNVLNYPGINHCVEITEGILVDECAALLCDFYRMPRQVLNAQKKAQSSINPSGSSGGSSGSVTPGTSESATPESSGGGFGGSAKNTITKTLQLRIVRPYNSAEVEKIVADEKNNREKIALEKNKDKVKEACSKHLKVAPYCTTQVERNACPFCKARKLDDKFYQKLRGQFPDAVFWQELGEILRQLQKQAAEIYNQSLIELYYEIFIKGRGFANASSVEHYLSDVCYTRAAELFKNAAIASGLRGKVKSNFRLKELKNMKSGLPTTKSDNFPIPLVKQKGGQYTGFEISSHNDDFIIKIPFGRWQVKKEINKYRPWEKFDFEQVRKSPKPISLLLSTQRRKRNKGWSKDEGTEAEIRKVMNGDYQTSYVEVKRGSKTGEKSAWMLNLSIDVPKIDKGVDPSIIGGIDVGVKSPLVCAINNAFSRYSISDNDLFRFNKKMFARRRILLKKNRHKRAGHGAKNKLKPISILTEKSKRFRKKLIERWACEIADFFIKNKVGTVQIENLESMKRKEDSYFNTRLRGFWPYAEMQNKIEFKLKQYGIEIKKVAPNNTSKTCSKCGHLNGYFNFEYRKKNKFPHFKCEKCNFKENADYNAALNISNPKLKSTKEEP

SEQ ID NO: 93 - protein, 726 aa, synthetic construct
SEVEFSHEYWMRHALTLAKRARDEREVPVGAVLVLNNRVIGEGWNRAIGLHDPTAHAEIMALRQGGLVMQNYRLIDATLYVTFEPCVMCAGAMIHSRIGRVVFGVRNNKHGAAGSLVNVLNYPGMTHRVEITEGILADECAALLCDFYRMPRQVFNARKKTQSSINPGGSSGGSSGSETPGTSESATPESSGGSSGSSAKNTITKTLKLRIVRPYNSAEVEKIVADEKNNREKIALEENKDKVKEACSKHLKVAAYCTTQVERNACLFCKARKLDDKFYQKLRGQFPDAVFWQEIGEIFRQLQKQAAEVYNQSLVELYYEILIKGKGIANASSVEHYLSDVCYTRAAELFKNAAIASGLRNKIKSNFRLKELRNMKSGLPTTKSDNFPIPLVRQKGGQYTGFEISNHDGDFIIKIPFGRWQVKKEINKYRPWEKFDFEQVRKSPKPISLLLSTQRRKRNKGWSKDEGTEAEIRKVMNGDYQTSYIEVKRGSKTGERSAWMLNLSIDVPKIDKGVDPSIIGGIDVGVKSPLVCAINNAFSRYSISDNDLFRFNKKMFARRRILLKKNKHKRAGHGAKNKLKPITIMTEKSKRFRKKLIERWACEIADFFIKNKVGTVQMENLESMKRKEDSYFNIRLRGFWPYAEMQNKIEFKLKQYGIEIRKVAPNNTSKTCSKCGHLNNYFNFEYRKKNKFPHFKCEKCNFKEDADYNAALNISNPKLKSTKEEP

SEQ ID NO: 94 - protein, 726 aa, synthetic construct
SEVEFSHEYWMRHALTLAKRARDEREVPVGAVLVLNNRVIGEGWNRAIGLHDPTAHAEIMALRQGGLVMQNYRLTDATLYVTFEPCVMCAGAMIHSRIGRVVFGVRNSKRGAAGSLMNVLNYPGMNHCVEITEGILVDECAALLCDFYRMPRQVLNAQKKARSCINPGGSSGGSSGSETPGTSESATPESSGGGSSGSAKNTITKTLQLRIVRPYNSAEVEKIVADEKNNRERIALEKNKDKVREACSKHLKVASYCTTQVERNACPFCKARKLDDKFYQKLRGQFPDAVFWQELGEILRQLQKQAAEIYNQSLIELYYEIFIKGKGFANASSVEHYLSDVCYTRAAELFKNAAIASGLRGKVKSNFRLKELKNMKSGLPTTKSDNFPIPLVKQKGGQYTGFEISSHNDDFIIKIPFGRWQVKEEIDKYRPWEKFDFEQVRKSPRPISLLLSTQRRKRNKGWSRDEGTEAEIKRVMNGDYQISYIEVKRGSKIGEKSAWMLSLSVDVPKIDKGVDPSIIGGIDVGVKSPLVCAINNAFSRYSISDNDLFRFNKKVFARRRILLKKNRHKRAGHGTKNKLKPITILTEKSGRFRRKLIERWACEIANFFIKNKVGTVQMENLESMKRKEDSYFNIRLRGFWPYAEMQNKIEFKLKQYGIKIRKVAPNNTSKTCSRCGHLNNYFSFEYRKKNKFPHFKCEKCNFKEDADYNAALNISNPKLKSTKEEP

SEQ ID NO: 95 - protein, 726 aa, synthetic construct
SEVEFSHEYWMRHALTLAKRARDEREVPVGAVLVQNNRVIGEGWNRAIGLHDPTAHAEIMALRQGGLVMQNYRLTDATLYVTFEPCVMCAGAMVHSRIGRVVFGVRNSKRGAAGSLMNVLNYPGMNHCVEITEGILVDECAALLCDFYRMPRQVLNAQKKAQSSISSGGSSGGSSGSETPGAGESVTPKSSVGSSAGSTKNTITKTLKLRIVRPYNSAEVEKIVADEKSNREKIALEKNRDKVKEACSKHLKVAAYCTTQVERNACLFCKARKLDDKFYQKLSGQFPDAVFWQELGGIFRQLQKQAAEIYNQSLIELYYEIFIKGKGITNASRVEHYLSDVCYTRAAELFKNAAIASGLRSKVRSNFRLKELKNMKSGLPTTKSDNFPIPLVKQKGGQYTGFEISSYNDDLIIKIPFGRWQVKKEIDKYRPWEKFDFEQVRKSPKPISLLLSTQRRKRNKGWSKDEGTEAEIRKVMNGDYQTSYIEVKRGSKIGEKSAWMLNLSINVPKIDKGVDPSIIGGIDVGVKSPLVCAINNALSRYSISDNDLFHFNKKMFARRRILLRKNRHKRAGHGAKNKLKPITMMTEKSKRFRKKLIERWACEIADFFIKNKVGTVQMENLESMKRKEDSYFNIRLRGFWPYAEMQDKIEFKLKQYGIVVRKVAPNNTSKTCSKCGHLNHYFNFEYRKKNKFPHFKCEKCNFKENADYNAALNISNPKLSSTKEEP

SEQ ID NO: 96 - protein, 726 aa, synthetic construct
SEVEFSHEYWMRHALTLAKRARDEREVPVGAILVLNNRVIGEGWNRAIGLHDPTAHAEIMALRQGGLVMQNYRLIDATLYVTFEPCVMCAGAMIHSRIGRVVFGVRNSKHGAAGSLVNVLNYPGMNHRVEITEGILADECAALLCDFYRMPRQVFNARKKAQSSINPSGSSGGSSGSVTPGTSESATPESSGGGFGGSAKNTITKTLQLRIVRPYNSAEVEKIVADEKNNREKIALEKNKDKVKEACSKHLKVASYCTTQVERNACLFCKARKLDDKFYQKLRGQFPDAVFWQEIGEIFRQLQRQAAEIYNQSLIELYYEIFIKGKGITNASRVEHYLSDVCYTRAAELFKNAAIASGLRNKVKSNFRLKELKNMKSGLPTTKSDNFPIPLVKQKGGQYAGFEISSHNDDFIIKIPFGRWQVKKEIDKYRPWEKFDFEQVRKSPKPISLLLSTRRRKRNKGWSKDEGTEAEIRKVMNGDYQTSYIEVKRGSKTGEKSAWMLNLSIDVPKIDKGVDPSIIGGIDVGVKSPLVCAINNAFSRYSISDNDLFRFNKKMFARRRILLKKNKHKRAGHGAKNKLKPISILTGKSERFRKKLIERWACEIADFFVKNKVGTVQMENLESMKRKEDSYFNIRLRGFWPYAEMQNRIEFKLKQYGIKVRKVAPNNTSKTCSKCGHLNSYFSFEYRKKNKFPHFKCEKCNFKENADYNAALNISNPKMKSTKEEP

SEQ ID NO: 97 - protein, 726 aa, synthetic construct
SEVEFSHEYWMRHALTLARRARDEREVPVGAILVLNNRVIGEGWNRAIGLHDPTAHAEIMALRQGGLVMQSYRLADATLYVTFEPCVMCAGAMIHSRIGRVVFGVRNSKHGAAGSLMNVLNYPGMNHRVEITEGILADECAALLCDFYRMPRRVFNAQKKAQSSISSGGSSGGSSGSGTPGASESVTPKSSVGSSAGSTKNTITKTLKLRIVRPYNSAEVEKIVADEKNNREKIALEKNKDKVKEACSKHLKVASYCTTQVERNACLFCKARKLDDKFYQKLRGQFPDAVFWQELGGIFRQLQKQAAEIYNQSLIELYYEIFIKGKGITNASRVEHYLSDVCYTRAAELFKNAAIASGLRGKVKSNFRLKELKNMKSGLPTTKSDNFPIPLVKQKGGQYTGFEISSHNDDFIIKIPFGRWQVKKEIDRYRPWEKFDFEQVRKSPKPISLLLSTQRRKRNKGWSKDEGTEAEIRKVMNGDYQTSYIEVKRGSKIGEKSAWMLSLSIDVPKIDKGVDPSTIGGIDVGVKSPLVCAINNAFCRYSISDNDLFHFNKKMFARRRILLKKSRHKRAGHGAKNKLKPISILTEKSKRFRKKLIERWACEIADFFIKNKVGTVQMENLESMKRKEDSYFNIRLRGFWPYAEMQNKIEFKLKQYGIEIRKVAPNNTSKTCSKCGHLNNYFNFEYRKKNKFPHFKCEKCNFKENADYNAALNISNPKLKSTKEEP

SEQ ID NO: 98 - protein, 726 aa, synthetic construct
SEVEFSHEYWMRHALTLAKRARDEREVPVGAVLVLNNRVIGEGWNRAIGLHDPTAHAEIMALRQGGLVMQNYRLTDATLYVTFEPCVMCAGAMIHSRIGRVVFGVRNSKRGAAGSLMNVLNYPGMNHCVEITEGILVDECAALLCDFYRMPRQVLSAQKKAQSSISPGGSSGGSSGSETPGASGSVTPKSSGGNSGGSAKNTITKTLKLRIVRPYNSAEVEKIVADEKNNRERIALEKNKDKVKEACSEHLKVAAYCTTQVERNACLFCKARKLDDKFYQKLRGQFPDAVFWQELGEIFRQLQKQTAEIYNQSLIELYYEIFIKGKGFANASSVEHYLSDVCYTRAAELFKNAAIASGLRGKVKSNFRLKELKNMKSGLPTTKSDNFPIPLVKQKGGQYTGFEISSHNDDFIIKIPFGRWQVKKEIDKYRPWEKFDFEQVRKSPKPISLLLSTQRRKRNKGWSKDEGTEAEIRKVMNGDYQTSYIEVKRGSKIGEKSAWMLNLSIDVPKIDKGVDPCIIGGIDVGVKSPLVCAINDAFSRYSISDNDLFHFNKKMFARRRILLKKNGHKRAGHGAKNKLKPITIMTEKSKRFRKKLIERWACEIADFFIKNKVGTVQMENLESMKRKEDSYFNIRLRGFWPYAEMQNKIEFKLKQYGIVVRKVAPNNTSKTCSKCGHLNNYFNFEYRKKNKFPHFKCEKCNFKENADYNAALNISNPQLKSTKGEP

SEQ ID NO: 99 - protein, 726 aa, synthetic construct
SEGEFSHEYWMRHALTLAKRARDEREVPVGAVLVLNNRVIGEGWNRTIGLHDPTAHAEIMALRQGGLVMQNYRLTDATLYVTFEPCVMCAGAMIHSRIGRVVFGVRNSKRGAAGSLMNVLNYPGMNHCVEITEGILVDECAALLCDFYRMPRQVLNAQKKAQSSISSGGSSGGSSGSEAPGASESVTPKSSGGSSGGSAKNTITKALKLRIVRPYNSAEVEKIVADEKNNRERIALEKNKDKVKEACSEHLKVAAYCTTQVERSACLFCKARKLDDKFYQKLRGQFPDAVFWQEIGEIFRQLQKQAAEIYNQSLIELYYEIFIKGRGFANASSVEHYLSDVCYTRAAKLFKNAAIASGLRGKVKSNFRLKELKNMKSGLPTTKSDNFPIPLVKQKGGQYTGFEISSHNDDFIIKIPFGRWQAKKEIDKYRPWEKFDFEQVRKSPKPISLLLSTQRRKRNKGWSKDEGTEAEIRKVMNGDYQTSYIEVKRGSKIGEKSAWMLNLSIDVPKIDKGVDPSIIGGIDVGVKSPLVCAINNALSRYSISDNDLFHFNKKMFARRRILLRKNRHKRAGHGAKNKLKPITIMTERSKRFRKKLIERWACEIADFFIKNKVGTVQMENLESMKRKEDSYFNVRLRGFWPYAEMQNKIEFKLKQYGIVVRKVAPNNTSKTCSKCGHLNNYFNFEYRKKNKFPHFKCEKCNFKEDADYNAALNISNPKLRSTKEEP

SEQ ID NO: 100 - protein, 726 aa, synthetic construct
SEVEFSHEYWMRHALTLAKRARDGREVPVGAVLVLNNRVIGEGWNRAIGLHDPTAHAEIMALRQGGLVMQNYRLIDATLYVTFEPCVMCAGAMVHSRIGRVVFGVRNGKRGAAGSLMNVLDYPGMGHRVEITEGILADECAALLCDFYCMPRQVFNAQKRAQSSINSGGSSGGNSGSETPGTSESATPGSSGGGSSGSAKNTITKTLQLRIVRPYNSAEVEKIVADEKNNRERIALEKNKDKVKEACSKHLKVASYCTTQVERNACPFCKARKLDDKFYQKLRGQFPDAVFWQELGEILRQLQKQAAEIYNRSLIELYYEIFIKGRGFANASSVEHYLSDVCYTRAAELFKNAAIASGLRGKVKSNFRLKELKNMKSGLPTTKSDNFPIPLVKQKGGQYTGFEISSHNDDFIIKIPFGRWQVKKEIDKYRPWEKFDFEQVRKSPKPISLLLSTQRRKRNKGWSKDEGTEAEIRKVMNGDYQTSYIEVKRGSKAGEKSAWMLNLSIDVPKIDKGVDPCIIGGIDVGVKSPLVCAINDAFSRYSISDNDLFHFNKKMFARRRILLKKNGHKRAGHGAKNKLKPITIMTEKSKRFRKKLIERWACEIADFFIKNKVGTVQMENLESMKRKEDSYFNIRLRGFWPYAEMQNKIEFKLKQYGIVVRKVAPNNTSKTCSKCGHLNNYFNFEYRKKNKFPHFKCEKCNFKEDADYNAALNISNPKLKSTKGEP

SEQ ID NO: 101 - protein, 726 aa, synthetic construct
SEVEFSHEYWMRHALTLAKRARDEREVPVGAVLVLNNRVIGEGWNRAIGLHDPTAHAEIMALRQGGLVMQNYRLIDATLYVTFEPCVMCAGAMIHSRIGRVVFGVRNNKRGAAGSLMNVLNYPGMNHRVEITEGILADECAVLLCDFYRMPRQVLNAQRKARSCIRSGGSSGGSSGSETPGASESVTPKSSGGSSAGSTKNTITKTLKLRIVRPYNSAEVEKIVADEKNSREKIALEKNKDKVKEACSKHLKVAAYCTTQVERNACLFCKARKLDDRFYQKLRGQFPDAVFWQEIGEIFRQLQKQAAEIYNQSLVELYYEIFIKGKGIANASSVEHYLSDVCYTRAAELFKNAAIASGLRNKIKSNFRLKELRNMKSGLPTTKSDNFPIPLVKQKGGQYTGFEISSHNDDFIIKIPFGRWQVKKEIDKYRPWEKFDFEQVRKSPKPISLLLSTQRRKRNKGWSKDEGTEAEIRKVMNGDYQTSYIEVKRGSRIGEKSAWMLSLSIDVPKIDRGVDPSIIGGIDVGVKSPLVCAINNGLSRYSISDNDLFHFNKKMFARRRILLKKNRHRRAGHGARNKLKPITVLTEKSKRFRKKLIERWACEIANFFVKNKVGTVQMENLESMKRKEDSYFNIRLRGFWPYAEMQSKIEFKLKQYGIKVRKVAPNNTSKTCSKCGHLNNYFNFEFRKKNKFPHFKCEKCNFKEDADYNAALNISNPKLKSTKEEP

SEQ ID NO: 102 - protein, 726 aa, synthetic construct
SEVEFSHEYWMRHALTLAKRARDGREVPVGAVLVLNNRVIGEGWNRAIGLHDPTAHAEIMALRQGGLVTQNYRLIDATLYVTFEPCAMCAGAMVHSRIGRVVFGVRNSKRGAAGSLMNVLNYPGMDHRVEITGGILADECAALLCDFYRMPRRVFNAQKKAQSSINSGGSSGGSSGSVTPGTSESATPESSGGGFGGSAKNTITKTLQLRIVRPYNSAEVEKIVADEKNNREKIALEKNKDKVKEACSKHLKVASYCTTQVERNACLFCKARKLDDKFYQKLRGQFPDAVFWQELGEIFRQLQKQAAEIYNQSLIELYYEIFIKGKGIANASSVEHYLSDVCYTRAAELFKNAAIASGLRNKIKSNFRLKELRNMKSGLPTTKSDNFPIPLVRQKGGQYTGFEISNHNGDFIIKIPFGRWQVKKEISKHRPWEKFDFEQVRKSPKPISLLLSTQRRKRNKGWGKDEGTEAEIRKVMNGDYQTSYIEVKRGSKIGEKSAWMLNLSIDVPKIDKGVDPSIIGGIDVGVKSPLVCAINNAFSRYSISDNDLFRFNKKMFARRRILLGKNRHKRAGHGVKNKLKPITILTEKSGRFRKKLIERWACEIADFFVKNKVGTVQMENLESMKRKEDSYFNIRLRGFWPYAEMQNKIEFKLKQYGIKVRKVAPNNTSKTCSKCGHLNNYFSFEYRKKNKFPHFKCEKCNFKENADYNAALNISNPKLKSTKEEP

SEQ ID NO: 103 - protein, 726 aa, synthetic construct
SEVEFSHEYWMRHALTLAKRARDEREVPVGAVLVLNNRVIGEGWNRAIGLHDPTAHAEIMALRQGGLVMQNYRLTDATLYVTFEPCVMCAGAMIHSRIGRVVFGVRNSKRGAAGSLMNVLDYRGMDHCVEITEGILVDECAALLCDFYRMPRQVLNAQKKAQSSISPGGSSGGSSGSETPGASGSVTPKSSGGSSAGSTKDTITKTLKLRIVRPYNSAEVEKIVADEKNSREKIALEKNKDKVKEACSKHLKVASYCTTQVERNACLFCKARKLDDKFYQKLRGQFPDAVFWQELGGIFRQLQKQAAEIYNQSLIELYYEIFIKGKGITNASRVEHYLSDVCYTRAAELFKNAAIASGLRSKVRSNFRLKELKNMKSGLPTTKSDNFPIPLVKQKGGQYTGFEISSHNSDFIIKIPFGRWQEKEEIDKYRPWEKFDFEQVRRSPKPISLLLSTQRRKKNKGWSKDEGTEAEIRRVMNGDYQTSYIEVKRGSKIGEKSAWMLNLSIDVPKIDKGVDPSIIGGIDVGVKSPLVCAINNALSRYSISDNDLFHFNKKMFARRRILLRKNRHKRAGHGAKNKLKPITIMTEKSKRFRKKLIERWACEIADFFIKNKVGTVQMENLESMKRKEDSYFNIRLRGFWPYAEMQSKIEFKLKQYGIVVRKVAPNNTSKTCSKCGHLNNYFNFEYRKKNKFPHFKCEKCNFKEDADYNAALNISNPKLKSTKGEP

SEQ ID NO: 104 - protein, 726 aa, synthetic construct
SEVEFSHEYWMRHALTLARRARDEREVPVGAILVLNNRVVGEGWNRAIGLHDPTAHAEIMALRQGGLVMQNYRLTDATLYVTFEPCVMCAGAMIHSRIGRVVFGVRNSKHGAAGSLVNVLNYPGMNHRVEITEGILADECAALLCDFYRMPRQVFNARKKAQSSIGPGGSSGGSGGSETPGTSESATLENSGGSSGGSAKNTITKTLKLRIVRPYNSAEVEKIVADEKNNREKIALEKNKDKVKEACSKHLKVASYCTTQVERNACLFCKARKLDDKFYQKLRGQFPDAVFWQELGEILRQLQKQAAEIYNQSLIELYYEIFIKGRGFANASSVEHYLSDVCYTRAAELFKNAAIASGLRGKVKSNFRLKELKNMKSGLPTTKSDNFPIPLVRQKGGKYTGFEISSHNDDFIIKIPFGRWQVKKEIDKYRPWEKFDFEQVRKSPKPISLLLSTQRRKRNKGWSKDEGTEAEIRKVMNGDYQTSYIEVKRGSRIGEKSAWMLSLSIDVPKIDRGVDPSIIGGIDVGVKSPLVCAINNALSRYSISDNDLFHFNKKMFARRRILLKKNRHRRAGHGARNKLKPITILTEKSGRFRKKLIERWACEIADFFIKNKVGTVQMENLESMKRKEDSYFNIRLRGFWPYAEMQNKIEFKLKQYGIVVRKVAPNNTSKTCSKCGHLNSYFNFEYRKKNKFPHFKCEKCNFKEDADYNAALNISNPKLKSTKEEP

SEQ ID NO: 105 - protein, 726 aa, synthetic construct
SEVEFSHEYWMRHALTLAKRARDEREVPVGAILVLNNRVIGVGWNRAIGLHDPTAHAEIMALRQGGLVMQNYRLIDATLYVTFEPCVMCAGAMIHSRIGRVVFGVRNSKHGAAGSLVNVLNYPGMNHRVEITEGILADECAALLCDFYRMPRQVFNARKKAQSSINSGGSSGGSSGSGTPGTSESATPKSSGGSSGGSAKNTITKTLKLRIVRPYNSAEVEKIVADEKNSREKIALEKNKDKVKEACSKHLKVAAYCTTQVERNACLFCKARKLDDKFYQKLRGQFPDAVFWQEIGEIFRQLQKQAAEIYNQSLIELYYEIFIKGKGFANASSVEHYLSDVCYTRAAELFKNAAIASGLRGKVKSNFRLKELKNMKSGLPTTKSDNFPIPLVKQKGGQYTGFEISSHNDDFIIRIPFGRWQVKEEIDKYRPWEKFDFEQVRKSPKPISLLLSTQRRKRNKGWSKDEGTEAEIRKVMNGDYQTSYIEVKRGSKTGEKSAWMLSLSIDVPKIDKGVDPSIIGGIDVGVKSPLVCAINNAFSRYSISDNDLFHFNKKMFARRRVLLKKSKHKRAGHGAKNKLKPITILTEKSGRFRKKLIERWACEIADFFVKNKVGTVQMENLESMKRKEDSYFNIRLRGFWPYAEMQNKIEFKLKQYGIKVRKVAPNNTSKTCSKCGHLNNYFSFEYRKKNKFPHFKCEKCNFKENADYNAALNISNPKLKGTKEEP

SEQ ID NO: 106 - protein, 727 aa, synthetic construct
SEVEFSHEYWMRHALTLAKRARDEREVPVGAVLVLNNRVIGEGWNRAVGLHDPTAHAEIMALRQGGLVMQNYRLTDATLYVTFEPCVMCAGAMIHSRIGRVVFGVRNSKRGAAGSLMNVLNYPGMNHCVEITEGILMDECAALLCDFYRMPRQVLNAQKKAQSSISSGGSSGGSSSSETPGASESVTPKSSVGSSAGSTKNTITKTLQLRIVRPYNSAEVEKIVADEKNNREKIALEKNKDKVREACSKHLKVASYCTTQVERNACPFCKARKLDDGFYQKLRGQFPDAVFWQEIGEIFRQLQKQAAEIYNQSLIELYYEIFIKGKGFANASSVEHYLSDVCYTRAAELFKNAAIASGLRGKVKSNFRLKELKNMKSGLPTTKSDNFPIPLVKQKGGQYTGFEISSHNDDLIVKIPFGRWQVKKEIDRYRPWEKFDFEQVRRSPKPISLLLSTQRRKRNKSWSKDEGTEAEIRKVMNGDYQTSYIEVRRGSKIGEKNAWMLSLSIDVPKIDKGVDPSIIGGIDVGVKSPLVCAINNAFSRYSISDNDLFRFNKKMFARRRILLKKNRHKRAGHGAKNKLKPITIMTEKSKRFRKKLIERWACEIADFFIKNKVGTVQMENLESMKRKEDSYFNIRLRGFWPYAEMQNKIEFKLKQYGIEIRKVAPNNTSKTCSKCGHLNNYFNFEYRKKNKFPHFKCEKCNFKENADYNAALNISNPKLKSTKEEPY

SEQ ID NO: 107 - protein, 726 aa, synthetic construct
SEAEFSHEYWMRHALTLARRARDEREVPVGAILVLNNRVIGEGWNRAIGLHDPTAHAEIMALRQGGLVLQNYRLVDATLYVTFEPCVMCAGAMIHSRIGRVVFGVRNSKRGAAGSLMNVLNYPGMNHCVEITEGILVDECAALLCDFYRMPRQVLHAQKKAQSSISPGGSSGGSSGSETPGASESVTPKSSGGSSGGSARNTITKTLKLRIIRPYNSAEVEKIVADEKDNRERIALEKNKGKVKEACSKHLKVASYCTTQVERNACLFCKARMLDDKFYQRLRGQFPDAVFWQELGEIFRQLQKQAAEIYNQSLIELYYEIFIKGKGFANASSVEHYLSDVCYTRAAGLFKNAAIASGLRGKVKSNFRLKELKNMKSGLPTTKSDNFPIPLVRQKGGQYTGFEISSHNDDFIIKIPFGRWQVRKEIDKYRPWEKFDFEQVRKSPKPISLLLSTQRRKRNKGWSKDEGTEAEIRKVMNGDYQTSYIEVKRGSKTGEKSAWMLNLSIDVPKIDKGVDPSIIGGIDVGVKSPLVCAINNAFSRYSISDNDLFHFNKKMFARRRILLKKNRHKRAGHGAKNKLKPISILTEKSKRFRKKLIERWACEIADFFIKNKVGTVQMENLESMKRREDSYFNIRLRGFWPYAEMQNKIEFKLKQYGIEIRKVAPNNTSKTCSKCGHLNNYFNFEYRKMNKFPHFKCEKCNFKENADYNAALNISNPKLKSTKEEP

SEQ ID NO: 108 - protein, 726 aa, synthetic construct
SEVEFSHEYWMRHALTLAKRARDEREVPVGAILVLNNRVIGEGWNRAIGLHDPTAHAEIMALRQGGLVMQNYRLIDATLYVTFEPCVMCAGAMIHSRIGRVVFGVRNSKHGAAGSLVNVLNYPGMNHRVEITEGILADECAALLCDFYRMPRQVLNAQKRARPCINSGGSSGGSGGSDTPSTSESTTPESSGGSSGGSAKNTITKTLKLRIVRPYNSAEVEKIVADEKDNREKIALEKNKGKVKEACSKHLKVAAYCTTQVERNACLFCKARKLDDKFYQELRGQFPDAVFWQELGGIFRQLQKQAAEIYNQSLIELYYEIFIKGKGITNASRVEHYLSDVCYTRAAELFKNAAIASGLRGKVKSNFRLKELKNMKSGLPTTKSDNFPIPLVKQKGGQYTGFEISSHNDDFIIKIPFGRWQAKKEIDKYRPWEKFDFEQVRKSPKPISLLLSTQRRKRNKGWSKDEGTEAEIRKVMNGDYQTSYIEVKRGSKTGEKSAWMLNLSIDVPKIDKGVDPSIIGGIDVGVKSPLVCAINNAFSRYSISDNDLFRFNKKVFARRRILLKRNGHKRAGHGTKNKLKPITTLTEKSGRFRKKLIERWACEIANFFIKNKVGTVQMENLESMKRKEDSYFNIRLRGFWPYAEMQNKIEFKLKQYGIKIRKVAPNNTSKTCSKCGHLNNYFSFEYRKKNKFPHFKCEKCNFKEDADYNAALNISNPKLKSTKEEP

SEQ ID NO: 109 - protein, 726 aa, synthetic construct
SEVEFSHEYWMRHALTLAKRARDEREVPVGAVLVLNNRVIGEGWNRAIGLHDPTAHAEIMALRQGGLVMQNYRLTDATLYVTFEPCVMCAGAMIHSRIGRVVFGVRNSRRGAAGSLMNVLNYPGMNHCVEITEGILMDECAALLCDFYRMPRQVLSAQKKAQSSISSGGPSGGSSCSETPGASESVTPKSSGGSSTGSTKNTITKTLKLRIVRPYNSAEVEKIVADEKNSREKIALEKNKDKVKEACSKHLKVASYCTTQVERNACPFCKARKLDDKFYQKLRGQFPDAVFWQELGEILRQLQKQAAEIYNQSLIELYYEIFIKGRGFANASSVEHYLSDVCYTRAAELFKNAAIASGLRNKIKSNFRLKELKNMRSGLPTTKSVNFPIPLVKQKGGQYTGFEVRNHNSDFIIKIPFGKWLVKKEINKYRPWEKFDFEQVRKSPKPISLLLSTQRRKRNKGWSKDEGTEAEIRKVMNGDYQISYIEVKRGRKIGEKSAWMLNLSIDVPKIDKGVDPSIVGGIDVGVKSPLVCAINSALGRYSISDNDLFHFNKKMFARRRILLKKNGHKRAGHGARNKLKPITVLTEKSKRFRKKLIERWACEIANFFIKNRVGTVQMENLESMKRKEDSYFNIRLRGFWPYAEMQNRIEFKLKQYGIEIRKVAPNNTSKTCSKCGHLNNYFNFEYRKKNKFPHFKCEKCNFKEDADYNAALNISNPKLKSTKEEP

SEQ ID NO: 110 - protein, 726 aa, synthetic construct
SEVEFSHEYWMRHALTLAKRARDEREVPVGAVLVLNNRAIGEGWNRAIGLHDPTAHAEIMALRQGGLVMQNYRLTDATLYVTFEPCVMCAGAMIHSRIGRVVFGVRNSKRGAAGSLMNVLNYPGMNHCVEITEGILVDECAALLCDFYRMPRQVLNAQKKAQSSISSGGSSGGSSGSETPGASGSVTPKSSGGSSAGSTKDTITKTLKLRIVRPYNSAEVEKVVADEKNNREKIAMEKNKDKVKEACSKHLKVASYCTTQVERNACLFCKARKLDDKFYQKLRGQFPDAVFWQEIGEIFRQLQRQAAEIYNQSLIELYYEIFIKGKGFANASSVEHYLSDVCYTRAAELFKNAAIASGLRGKVKSNFRLKELKNMKSGLPTTKSDNFPIPLVKQKGGQYTGFEISSHNDDFIIKIPFGRWQVKKEIDKYRPWEKFDFEQVRKSPKPISLLLSTQRRKRNKGWSKDEGTEAEIRKVMNGDYQTSYIEVKRGSKVGEKSAWMLSLSIDVPKIDKGVDPSIIGGIDVGVRSPLVCAINNAFSRYSISDNDLFHFNKKMFARRRILLKKNRHRRAGHGAKNKLKPITVLTEKSKRFRKKLIERWACEIANFFIKNKVGTVQMENLESMKRKEDSYFNIRLRGFWPYAEMQNKIEFKLKQYGIEIRKVAPNNTSRTCSKCGHLNNYFSFEYRKKNKFPHFKCEKCNFKEDADYNAALNISNPKLKSTKEEL

SEQ ID NO: 111 - protein, 726 aa, synthetic construct
SEVEFSHEYWMRHALTLAKRARDEREVPVGAVLVLNNRVIGEGWNRAIGLHDPTAHAEIMALRQGGLVMQNYRLTDATLYVTFEPCVLCAGAMVHSRIGRVVFGVRNSKRGAAGSLMNVLNYPGMNHRVEITEGILADECAALLCDFYRMPRQVFNAQKKARSNISSGGSSGGSSGSETPGTSESATPEGSGGNSGGSAKNTITKTLKLRIVRPYNSAEVEKIVADEKNNREKIALEKNKGKVKEACSEHLKVAAYCTTQVERNACLFCKARKLDDKFYQKLRGQFPDAVFWQELGEILRQLQKQAAEIYNQSLIELYYEIFIKGKGFANASSVEHYLSDVCYTRAAELFKNAAIASGLRGKVKSNFRLKELKNMKSGLPTTKSDNFPIPLVKQKGGQYTGFEISSHNDDFIIKIPFGRWQVKEEIDKYRPWEKFDFEQVRKSPKPISLLLSTQRRKRNKGWSKDEGTEAEIRKVMNGDYQTSYIEVKRGSKIGEKSAWMLNLSIDVPKIDKGVDPNIIGGIDVGVKSPLVCAISNAFSRYSISDNDLFHFNKKMFARRRILLKKSKHKRAGHGAKNKLKPITILTEKSRRFRKKLIERWACEIADFFIKNKVGTVQMENLESMKRREDSYFNIRLRGFWPYAEMQNKIEFKLKQYGIKIRKVAPNNTSRTCSECGHLNNYFNFEYRKKNKFPHFKCEKCNFKENADYNAALNISNPKLKSTKEEP

SEQ ID NO: 112 - protein, 726 aa, synthetic construct
SEVEFSHEYWMRHALTLAKRARDEREVPVGAILVLNNRVIGEGWNRAIGLHDPTAHAEIMALRQGGLVMQNYRLIDATLYVTFEPCVMCAGAMIHSRIGRVVFGVRNNKHGAAGSLVNVLNYPGMNHRVEITEGILADECAALLCDFYRMPRQVFNARKKAQSSINSGGSSGGSSGSVTPGTSESATPESSGGSSGGSAKNTITKTLKLRIVRPYNSAEVEKIVADEKNNREKIALEKNKDKVKEACSEHLKVAAYCTTQVERNACLFCKARKLDDKFYQKLRGQFPDAVFWQEIGEIFRQLQRQAAEIYNQSLIELYYEIFIKGRGFANASSVEHYLSDVCYTRAAELFKNAAIASGLRGKVKSNFRLKELKNMKSGLPTTKSDNFPIPLVKQKGGQYTGFEISNHNGDFIIKIPFGRWQAKKEIDKYRPWEKFDFEQVRKSPKPISLLLSTQRRKRNKGWSKDEGTEAEIRKVMSGDYQTSYIEVKRGSKIGEKSTWMLNLSIDVPKIDKGVDPSIVGGIDVGVKSPLVCAINNSFSRYSICDNDLFRFNKKMFARRRILLKKSKHKRAGHGAKNKLKPITILTEKSRRFRKKLIERWACEIADFFIKNKVGTVQMENLESMKRKEDSYFNIRLRGFWPYAEMQNKIEFKLKQYGIEIRKVAPNNTSKTCSKCGHLNNYFNFEYRKKNKFPHFKCEKCNFKENADYNAALNISNPKLKSTKEKP

SEQ ID NO: 113 - protein, 726 aa, synthetic construct
SEVEFSHEYWMRHALTLAKRARDEREVPVGAVLVLNNRVIGEGWNRAIGLYDPTAHAEIMALRQGGLVMQNYRLTDATLYVTFEPCVMCAGAMIHSRIGRVVFGVRNSKRGAAGSLMNVLNYPGMNHCVEITEGILVDECAALLCDFYRMPRQVLNAQKKAQPSINPGGSSGGSSGSETPGTSESATPESSGGSSGGSAKNTITKTLKLRIVRPYNSAEVEKIVADEKNNRERIALEKNKDKVKEACSEHLKVAAYCTTQVERNACLFCKARKLDDKFYQKLRGQFPDAVFWQELGGIFRQLQKQAAEIYNQSLIELYYEIFIKGKGITNASRVEHYLSDVCYTRAAELFKNAAIASGLRSKVRSNFRLKELKNMKSGLPTTKSDNFPIPLVKQKGGQYTGFEISSHNSDFIIKIPFGRWQEKEEIGKYRPWEKFDFEQVRRSPKPISLLLSTQRRKKNKGWSKDEGTEAEIRRVMNGDYQTSYIEVKRGSKIGEKSAWMLNLSIDVPKIDKGVDPSIIGGIDVGVKSPLVCAINNSSSRYSICDNDLFRFNKKMFARRRILLKKNRHKRAGHGAKNKLKPITILTEKSGRFRKKLIERWACEIANFFIKNKVGTVQMEDLESMKRKEDSYFNIRLRGFWPYAEMQNKIEFKLKQYGIKIRKVAPNNTSKTCSKCGHLNNYFSFEYRKKNKFPHFKCEKCNFKEDADYNAALNISNPKLKGTKEEP

SEQ ID NO: 114 - protein, 726 aa, synthetic construct
SEVEFSHEYWMRHALTLAKRARDEREVPVGAILVLNNRVIGEGWNRAIGLHDPTAHAEIMALRQGGLVMQNYRLIDATLYVTFEPCVMCAGAMIHSRIGRVVFGVRNNKHGAAGSLVNVLNYPGMNHRVEITEGILADECAALLCDFYRMPRQVFNARKRAQSSINPGGSSGGSSGSVTPGTGESATPKSTGGSSGGSAKNTITKTLKLRIVRPYNSAEVEKIVADEKNNREKIALEKNKGKVKEACSKHLEVAAYCTTQVERNACLFCKARKLDDKFYQKLRGQFPDAVFWQELGEIFRQLQRQAAEIYNQSLIELYYEIFIKGKGFANASSVEHYLSDVCYTRAAELFKNAAIASGLRGKVKSNFRLKELKNMKSGLPTTKSDNFPIPLVKQKGGQYTGFEISSHNDDFIIKIPFGRWQVKKEIDKYRPWEKFDFEQVRKSPKPISLLLSTQRRKRNKGWSKDEGTEAEIRKVMNGDYQTSYIEVKRGSKTGEKSAWMLNLSIDVPKIDKGVDPSIIGGIDVGVKSPLVCAINNAFSRYSISDNDLFRFNKKMFARRRILLRKNRHKRAGHGAKNKLKPISILTGKSERFRKKLIERWACEIADFFIKNKVGTVQMENLESMKRKEDSYFNIRLRGFWPYAEMQNKIEFKLKQYGIEIRKVAPNNTSKTCSKCGHLNNYFNFEYRKKNKFPHFKCEKCNFKENADYNAALNISNPKLKSTKEEP

SEQ ID NO: 115 - protein, 726 aa, synthetic construct
SEVEFSHEYWMRHALTLAKRARDECEVPVGAVLVLNNRVIGEGWNRAIGLHDPTAHAEIMALRQGGLVMQNHRLVDATLYVTFEPCVLCAGAMVHSRIGRVVFGVRNSKRGAAGSLMNVLNYPGMNHRVEITEGILADECAALLCDFYRMPRQVFNAQKKARSNTNSGDSSGGSSGSGIPGTSESATPESSGGSSGGSAKNTITKTLKLRIVRPYNSAEVEKIVADEKDNRERIALEKNKGKVKEACSKHLKVASYCTTQVERNACLFCKARRLDDKFYQKLRGQFPDAVFWQEIGEIFRQLQKQAAEVYNQSLVELYYEILIKGKGFANASSVEHYLSGVCYTRAAELFKNAAIASGLRGKVKSNFRLKELKNMRSGLPTTKSDNFPIPLVKQKGGQYTGFEISSHNDDFIIKIPFGRWQVKKEIDKYRPWEKFDFEQVRKSPKPISLLLSTQRRKRNKGWSKDEGTEAEIRKVMNGDYQTSYIEVKRGRKIGEKSVWMLNLSIDVPKIDKGVDPSTIGGIDVGVKSPLVCAINNAFSRYSISDNDLFRFNKKMFARRRILLKKNRHKRAGHGAKNKLKPITILTEKSGRFRKKLIERWACEIADFFIKNKVGTVQMENLESMKRKEDSYFNIRLRGFWPYAEMQNKIELKLKQYGIKIRKVAPNNTSKTCSKCGHLNDYFNFEYRKKNKFPHFKCEKCNFKEDADYNAALNISNPKLKSTREEP

SEQ ID NO: 116 - protein, 726 aa, synthetic construct
SEVEFSHEYWMRHALTLAKRARDEREVPVGAVLVLDNRVIGVGWNRAIGLHDPTAHAEIMALRQGGLVMQNYRLTDATLYVTFEPCVMCAGAMVHSRIGRVVFGVRNSKRGAAGSLMNVLNYPGMSHCVEITEGILVDECAALLCDFYHMPRQVLNAQKKAQSSISSGGSSGGSGGGETPGASESVTPKSSGGSSAGSTKNTITKTLKLRIVRPYNSAEVEKIVADEKNSREKIALEKNKDKVKEACSEHLKVAAYCTTQVERSACLFCKARKLDDRFYQKLRGQFPDAVFWQELGEILRQLQKQAAEIYNQSLIELYYEIFIKGRGFANAGSVEHYLSDVCYTRAAELFKNAAIASGLRGKVKSNFRLKELKNMKSGLPTTKSDNFPIPLVKQKGGQYTGFEISSHNDDFIIKIPFGRWQVKKEIDKYRPWEKFDFEQVRKSPKPISLLLSTQRRKRNKGWSKDEGTEAEIRKVMNGDYQTSYIEVKRGSKTGEKSAWMLNLSIDVPKIDKGVDPSIIGGIDVGVKSPLVCAINNAFSRYSISDNDLFRFNKKMFARRRILLKKNRHKRAGHGAKNKLKPISILTGKSGRFRKKLIERWACEIADFFIKNKVGTVQMENLGSMKRREDSYFNIRLRGFWPYAEMQNKIEFKLKQYGIEIRKVAPNNTSKTCSKCGHLNNYFNFEYRKKNKFPHFKCEKCNFKENADYNAALNISNPKLRSAKEEP

SEQ ID NO: 117 - protein, 726 aa, synthetic construct
SEVEFSHEYWMRHALTLAKRARDEREVPVGAVLVLNNRVIGEGWNRAIGLHDPTAHAEIMALRQGGLVMQNYRLTDATLYVTFEPCVMCAGAMIHSRIGRVVFGVRNSKRGAAGSLMNVLNYPGMNHCVEITEGILMDECAALLCDFYRMPRQVLSAQKKAQSSISSGGPSGGSSCSETPGASESVTPKSSGGSSTGSTKNTITKTLKLRIVRPYNSAEVEKIVADEKNSREKIALEKNKNKVKEACGKHLKMASYCTTQVERNACLFCKARKLDDKFYQKLRGQFPDAVFWQEIGEIFRQLQKQAAEVYNQSLVELYYEILIKGKGIANASSVEHYLSDVCYTRAAELFKNAAIASGLRNKIKSNFRLKELKNMKSGLPTTKSDNFPIPLVKQKGGQYTGFEISSHNDDFIIKIPFGRWQMKKEIDRYRPWEKFDFEQVRKSPKPISLLLSTQRRKRNKGWSKDEGTEAEIRRVMNGDYQTSYIEVKRGSKIGEKSAWMLSLSIDVPKIDKGVDPSIIGGIDVGVKSPLVCAINNAFCRYSISDNDLFHFNKKMFARRRILLKKSRHKRAGHGAKNKLKPISILTEKSKRFRKKLIERWACEIADFFIKNKVGTVQMENLESMKRKEDSYFNIRLRGFWPYAEMQNKIEFKLKQYGIEIRKVAPNNTSKTCSKCGHLNNYFNFEYRKKNKFPHFKCEKCNFKENADYNAALNISNPKLKSTKEEP

SEQ ID NO: 118 - protein, 726 aa, synthetic construct
SEVEFSHEYWMRHALSLAKRARDEREVPVGAVLVLNNRIIGEGWNRAIGLHDPTAHAEIMALRQGGLVMQNYRLTDATLYVTFEPCVMCAGAMVHSRIGRVVFGVRNSKRGAAGSLMNVLNYPGVNHCVEITEGILVDECAALLCDFYRMPRQVLNAQKKAQSSISPGGSSGGSSGSETPGASESVTPKSSGGSSGGSAKNTITKTLKLRIVRPYNSAEVEKIVADEKNNREKIALEKNKGKVKEACSKHLEVAAYCTTQVERNACLFCRARKLDDKFYQKLRGQFPDAVFWQELGEIFRQLQKQAAEIYNQSLIELYYEIFIKGKGFANASSVEHYLSDVCYTRAAELFKNAAIASGLRGKVKSNFRLKELKNMKSGLPTTKSDNFPIPLVKQKGGQYTGFEISNHNSDFIIKIPFGRWQVKKEINKYRPWEKFDFEQVRKSPKPISLLLSTQRRKRNKGWSKDEGTEAEIRKVMNGDYQTSYIEVKRGSRIGEKSAWMLSLSIDVPKIDRGVDPSIIGGIDVGVKSPLVCAINNALSRYSISDNDLFHFNKKMFARRRILLKKNRHKRAGHGAKNKLKPISIMTEKGKRFRKKLIERWACEIADFFIKNKVGTVQMENLESMKRKEDSYFNIRLRGFWPYAEMQNKIEFKLKQYGIEIRKVAPKNTSKTCSRCGHLNNYFSFEYRKKNKFPHFKCEKCNFKENADYNAALNISNPKLKSTKEEP

SEQ ID NO: 119 - protein, 726 aa, synthetic construct
SEVELSHEYWMRHALTLAKRARDEREVPVGAVLVLNNRVIGEGWNRAIGLHDPTAHAEIMALRQGSLVMQNYRLIDATLYVTFEPCVMCAGAMIHSRIGRVVFGVRNSKHGAAGSLVNVLNYPGMNHRVEVTEGILADECAALLCDFYRMPRQVFSARRKAQSSINPGGSFGGGSGSETPGASESATPESSGGSSGGSAKNTITKTLQLRIVRPYNSAEVERIVTDEKNNREKIALEKNKDKVKEACSRHLKMASYCTTQVERNACLFCKARKLDDKFYQKLRGQFPDAVFWQELGGIFRQLQKQAAEIYNQSLIELYYEIFIKGKGITNASRVEHYLSDVCYTRAAELFKNAAIASGLRNKIKSNFRLKELRNMKSGLPTTKSDNFPIPLVRQKGGQYTGFEISNHNGDFIIKIPFGRWQVKKEIDKYRPWEKFDFEQVRKSPKPISLLLSTQRRRRNKGWSKDEGTEAEIRKVMNGDYQTSYIEVKRGSKIGEKSAWMLSLSIDVPKIDKGVDPSIIGGIDVGVKSPLVCAINNALSRYSISDNDLFHFNKKMFARRRILLKKNRHKRAGHGAKNKLKPITILTKKSERFRKKLIERWACEIANFFVKNKVGTVQMENLESMKRKEDSYFNIRLRGLWPYAEMQNKIEFKLKQYGIEIRKVAPNNTSKTCSKCGHLNNYFNFEYRKRNKFPHFKCEKCNFKENADYNAALNISNPKLKGTKEEP

SEQ ID NO: 120 - protein, 726 aa, synthetic construct
SEVEFSHEYWMRHALTLAKRARDEREVPVGAVLVLNNRVIGEGWNRAIGLHDPTAHAEIMALRQGGLVMRNYRLTDATLYVTFEPCVMCAGAMIHSRIGRVVFGVRNNKHGAAGSLVNVLDYPGMNHRVEITEGILADECAALLCDFYRMPRQVFNARKKAQSSISPGGSSGGSSGSETPGASESVTPKSSGGSSAGSTKNTITKTLKLRIVRPYNSAEVEKIVSDEKNNRERIALEKNKDKVKEACSKHLKMAAYCTTQVERNACLFCKARRLDDKFYQKLRDQFPDAVFWQEIGEIFRQLQKQAAEIYNQSLIELYYEIFIKGRGFANAGSVEHYLSDVCYTRAAELFKNAAIASGLRGKVKSNFRLKELKNMKSGLPTTKSDNFPIPLVKQKGGQYTGFEISSHNDDFIIKIPFGRWQVKKEIDKYRPWEKFDFEQVRKSPKPISLLLSIQRRKRNKGWSKDEGTEAEIRKVMNGDYQTSYVEVKRGSKTGEKSAWMLNLSIDVPKIDKGVDPSIIGGIDVGVKSPLVCAINNAFSRYSISDNDLFRFNKKMFARRRILLKKNRHKRAGHGAKNKLKPISILTEKSKRFRKKLIERWACEIADFFIKNKVGTVQMENLESMKRKEDSYFNIRLRGFWPYAEMQNKIEFKLKQYGIEIRRVAPNNTSRTCSKCGHLNNYFNFEYRRKYKFPHFKCEKCNFKEDADYNAALNISNPKLKSTKEEP

SEQ ID NO: 121 - protein, 726 aa, synthetic construct
SEVEFSHEYWMRHALTLAKRARDEREVPVGAVLVLNNRVIGEGWNRAIGLHDPTAHAEIMALRQGGLVMQNYRLIDATLYVTFEPCVMCAGAMVHSRIGRVVFGVRNSKRGAAGSLMNVLNYPGMNHCVEITEGILVDECAALLCDFYRMPRQVLSAQKKAQSSVSSGGSSGGSSGSETPGASGSVTPKSSGGSSTGSTKNTITKTLKLRIVRPYNSAEVEKIVADEKNNREKIALEKNKDKVKEACSKHLKVASYCTTQVERNACPFCKARKLDDKFYQKLRGQFPDAVFWQELGEILRQLQKQAAEIYNQSLIELYYEIFIKGKGITNASRVEHYLSDVCYTRAAELFKNAAIASGLRSKVRSNFRLKELKNMKSGLPTTKSDNFPIPLVKQKGGQYTGFEISSHNDDFIIKIPFGRWQVKKEIDKYRPWEKFDFEQVRKSPKPISLLLSTQRRKRNKGWSKDEGTEAEIRKVMNGDYQTSYIEVKRGSKIGEKSAWMLNLSIDVPKIDKGVDPSIIGGIDVGVKSPLVCAVNNALSRYSISDNDLFHFNKKMFARRRILLKKNRHKRAGHGAKNKLKPITILTEKSGRFRKKLIERWACEIANFFIKNKVGTVQMENLESMKRKEDSYFNIRLRGFWPYAEMQNKIEFKLKQYGIKIRKVAPYNTSKTCSKCGHLNNYFSFEYRKKNKFPHFKCEKCSFKEDADYNAALNISNPRLKSTKEEP

SEQ ID NO: 122 - protein, 726 aa, synthetic construct
SEVEFSHEYWMRHALTLAKRARDEREVPVGAVLVLNNRVIGEGWNRAIGLHDPTAHAEIMALRQGGLVMQNYRLTDATLYVTFEPCVMCAGAMIHSRIGRVVFGVRNSKRGAAGSLMNVLNYPGMNHCVEITEGILVDECAALLCDFYRMPRQVLNAQKKAQSSISSGGSSGGSSGSETPGASESATPKSSGGSSAGSTKNTITKTLKLRIVRPYNSAEVEKIVADEKNNRERIALEKNKDKVKEACSKHLKVAAYCTTQVERNACLFCKARKLDDKFYQKLRGQFPDAVFWQETGEIFRQLQRQAAEIYNQSLIELYYEIFIKGKGFANASSVEHYLSDVCYTRAAELFKNAAIASGLRGKVKGNFRLKELKNMKSGLPTTKSDNFPIPLVKQKGGQYTGFEISSHNDDFIIKIPFGRWQAKKEIDKYRPWEKFDFEQVRKSPKPISLLLSTQRRKRNKGWSKDEGTEAEIRKVMNGDYQTSYIEVKRGSKIGEKSAWMLNLSIDVPKIDKGVDPSIIGGIDVGVKSPLVCAINDALSRYSISDNDLFHFNKKMFARRRILLRKNRHKRAGHGARNKLKPITVLTEKSERFRKKLIERWACEIANFFIKNKVGTVQMENLESMKRREDSYFNIRLRGFWPYAEMQSKIEFKLKQYGIEVRKVAPNNTSKTCSKCGHLNNYFNFEYRKMNKFPHFKCEKCNFKENADYNAALNISNPKLKSTKEEP

SEQ ID NO: 123 - protein, 726 aa, synthetic construct
SEVEFSHEYWMRHALTLAKRARDEREVPVGAVLVLNNRVIGEGWNRAIGLHDPTAHAEIMALRQGGLVMQNYRLIDATLYVTFEPCVMCAGAMIHSRIGRVVFGVRNSKHGAAGSLVNVLNYPGMNHRVEITEGILADECAALLCDFYRMPRQVFSARKKAQSSINSGGSSGGNSGSKTPGTSESATPESSGGSSGGPAKNTITKTLKLRIVRPYNSAEVEKIVADEKNNREKIALEKNKDKVKEACSKHLKVAAYCTTQVERNACQFCKARKLDDKFYQKLRGQFPDAVFWQEIGEIFRQLQKQAAEIYNQSLIELYYEIFIKGKGFANASSVEHYLSDVCYTRAAELFKNAAIASGLRGKVKSNFRLKELRNMKSGLPTTKSDNFPIPLVRQKGGQYTGFEISNHDGDFIIKIPFGRWQVKKEIDKYRPWEKFDFEQVRKSPKPISLLLSTQRRKRNKGWSKDEGTEAEIRKVMNGDYQTSYIEVKRGSRIGEKSAWMLSLSIDVPKIDRGVDPSIIGGIDVGVKSPLVCAINNALSRYSISDNDLFHFNKKMFARRRILLKKNRHKRAGHGAKNKLKPISILTEKSKRFRKKLIERWACEIADFFIKNKVGTVQMENLESMKRKEDSYFNIRLRGFWPYAEMQNRIEFKLKQYGIEIRKVAPNNTSKTCSKCGHLNNYFNFEYRKKNKFPHFKCEKCNFKENADYNAALNISNPKLKSTKEEP

SEQ ID NO: 124 - protein, 726 aa, synthetic construct
SEVEFSHEYWMRHALTLAKRARDEREVPVGAVLVLNNRVIGVGWNRAIGLHDPTAHAEIMALRQGGLVMQNYRLIDATLYVTFEPCIMCAGAMIHSRIGRVVFGVRNNKHGAAGSLVNVLNYPGMNHRVEITEGILADECAALLCDFYRMPRQVFNARKKAQSSINPGGSSGGSSGSETPGTSESATPESSGGSSGSSAKNTITKTLKLRIVRPYNSAEVEKIVADEKNNREKIALEKNKDKVKEACSKHLKMASYCTTQVERNACLFCKARKLDDKFYQKLRDQFPDAVFWQEIGEIFRQLQRQAAEIYNQSLIELYYEIFIKGKGFANASSVEHYLSDVCYTRAAELFKNAAIASGLRGKVKSNFRLKELKNMKSGLPTTKSDNFPIPLVKQKGGQYTGFEISSHNDDFIIKIPFGRWQVKEEIDKYRPWEKFDFEQVRKNPKPISLLLSIQRRKRNKGWSKDEGTEAEIKKVMNGDYQTSYIEVKRGSKIGEKSTWMLNLSIDVPKIDRGVDPSIIGGIDVGVKSPLVCAINNAFSRYSISDNDLFRFNKKMFARRRILLKKNRHKRAGHGAKNKLKPITILTGKSVRFRKKLIERWACEIADFFIKNKVGTVQMENLESMKRREDSYFNIRLRGFWPYAEMQSKIEFKLKQYGIEIRKVAPNNTSKTCSKCGHLNDYFNFEYRKKNKFPHFKCEKCNFKENADYNAALNISNPKLKSTKGEP

SEQ ID NO: 125 - protein, 726 aa, synthetic construct
SEVEFSHEYWMRHALMLAKRARDEREVPVGAVLVLNNRVIGEGWNRAIGLHDPTAHAEIMALRQGGLAMQNYRLVDATLYVTFEPCVLCAGAMVHSRIGRVVFGVRNSKRGAAGSLMNVLNHPGMNHRVEITGGILADECAALLCDFYRMPRQVFNAQKKARSNINSGGSSGGSSGSETLGTSESATPESSGGGSSGSAKNTITKTLKLRIVRPYNSAEVERIVADEKNNREKIALEKNKDKVKEACSKHLKVATYCTTQVERNACLFCKARRLDDKFYQKLRGQFPDAVFWQEIGEIFRQLQKQAAEIYNQSLVELYYEILIKGKGIANAGSVEHYLSDVCYTRAAELFKNAAIASGLRNKIKSNFRLKELRNMRSGLPTTKSDNFPIPLVRQKGGQYTGFEINNHNGDFIIKIPFGRWQVKKEINKHRPWEKFDFEQVRKSPKPISLLLSTQRRKRNKGWSKDEGTEAEIRKVVNGDYQTSYIEVKRGSKIGEKSAWMLNLSIDVPKIDKGVDPSIIGGIDVGVKSPLVCAINNAFSRYSISDNDLFHFNKKMFARRRILLRKNRHRRAGHGAKNKLKPITILTEKSKRFRKKLIERWACEIADFFIKNKVGTVQMENLESMKRKEDSYFNIRLRGFWPYAEMQNKIEFKLKQYGIKIRKVAPNNTSRTCSKCGHLNNYFSFEYRKKNKFPHFKCEKCNFKEDADYNAALNISNPKLKGTKEEL

SEQ ID NO: 126 - protein, 726 aa, synthetic construct
SEVEFSHEYWMRHALTLAKRARDEREVPVGAILVLNNRVIGEGWNRAIGLHDPTAHAEIMALRQGGLVMQNYRLTDATLYVTFEPCVMCAGAMIHGRIGRVVFGVRNNKHGAAGSLVNVLNYPGMNHRVEITEGILADECAALLCDFYRMPRQVFNARKKAQSSISPGGSSGGSSGSETPGTSESVTPKSSGGSSGGSAKNTITKTLKLRIVRPYNSAEVEKIVADEKNNREKIALEKNKGKVKEACSKHLKVASYCTTQVERNACLFCKARKLDDKFYQKLRGQFPHAVFWQELGEIFRQLQKQAAEIYNQSLIELYYEIFIKGRGFANASSVEHFLSDVCYTRAAELFKNAAIASGLRGKVKSNFRLKELKNMRSGLPTTKSDNFPIPLVKQKGGQYTGFEISSHNDDFIIKIPFGRWQVKKEIDKYRPWEKFDFEQVRKSPKPISLLLSTQRRKRNKGWSKDEGTEAEIRKVMNGDYQTSYIEVKRGSKTGEKSAWMLNLSIDVPKIDKGVDPSIIGGIDVGVKSPLVCAINNASSRYSISDNDLFHFNKKMFARRRILLKKNRHKRAGHGVKNKLKPISILTEKSKRFRKKLIERWACEIADFFIKNKVGTVQMENLESMKRKEDSYFNIRLRGFWPYAEMQNKIEFKLKQYGIEIRKVAPNNTSKTCSKCGHLNNYFNFEYRKKNKFPHFKCEKCSFKENADYNAALNISNPKLKSTKEEP

SEQ ID NO: 127 - protein, 726 aa, synthetic construct
SEVEFSHEYWMRHALTLAKRARDEREVPVGAVLVLNNRVIGVGWNRAIGLHDPTAHAEIMALRQGGLVMQNYRLTDATLYVTFEPCVMCAGAMIHSRIGRVVFGVRNSKRGAAGSLMNVLNYPGMNHCVEITEGILVDECAALLCDFYRMPRQVLNAQKKAQSSISSGGSSGGSSGSETPGASGSVTPKSSGGSSAGSTKDAITKTLKLRIVRPYNSAEVEKVVADEKNNREKIALEKNRDKVKEACSEHLKVAAYCTTQVERNACLFCKARKLDDKFYQKLRGQFPDAVFWQELGGIFRQLQKQAAEIYNQSLIELYYEIFIKGKGITNASRVEHYLSDVCYTRAAELFKNAAIASGLRSKVRSNFRLKELKNMKSGLPTTKSDNFPIPLVKQKGGQYTGFEISSHNSDFIIKIPFGRWQVKKEIDKYRPWEKFDFAQVRKSPKPISLLLSTQRRKRNRGWSKDEGTEAEIKKVMNGDYQTSYIEVKRGSKIGEKSAWMLNLSINVPKIDKGVDPSIIGGIDVGVKTPLVCAINNAFSRYSISDNDLFHFNKKMFARRRILLKKSKHKRAGHGAKNKLKPITILTEKSKRFRKKLIERWACEIADFFIKNKVGTVQMENLESMKRKEDSYFNIRLRGFWPYAEMQDKIEFKLKQYGIEIRKVAPNNTSKTCSRCGHLNNYFNFEYRRKNKFPHFKCEKCNFKENADYNAALNISNPKLKSTKEEP

SEQ ID NO: 128 - protein, 726 aa, synthetic construct
SEVEFSHEYWMRHALTLAKRARDEREVPVGAILVLNNRVIGVGWNRAVGLHDPTAHAEIMALRQGGLVMQNYRLVEATLYVTFEPCIMCAGAMIHSRIGRVVFGVRNSKRGAAGSLMNVLNYPGMNHRVEITEGILADECAALLCDYYRMPRQVFNARKKAQSSINSGGSSDGGSGSETPGTSESATPESSGGSSGGSAKNTITKTLKLRIVRPYNSAEVEKIVADEKNNREKIALEKNKDKVKEACSEHLKVAAYCTTQVERSACLFCKARKLDDKFYQKLRGQFPDAVFWQELGEILRQLQKQAAEIYNQSLIELYYEIFIKGRGFANASSVEHYLSDVCYTRAAELFKNAAIASGLRGKVKSNFRLKELKNMKSGLPTTKSDNFPIPLVKQKGGQYTGFEISSHNDDFIIKIPFGRWRVKKEIDKYRPWEKFDFEQVRKSPKPISLLLSTQRRKRNKGWSKDEGTEAEIRKVMNGDYQTSYIEVKRGSKIGEKSAWMLNLSIDVPKIDKGVDPSIIGGIDVGVKSPLVCAINNAFSRYSISDNDLFHYNKKMFARRRILLKKNRHKRAGHGAKNKLKPITILTEKSRRFRKKLIERWACEIADFFVKNKVGTVQMENLESMKRKEDSYFNIRLRGFWPYAEMQNKIEFKLKQYGIEIRKVAPNNTSKTCSKCGHLNNYFNFEYRKKNKFPHFKCEKCNFKENADYNAALNISNPKLKSTKEEP

SEQ ID NO: 129 - protein, 726 aa, synthetic construct
SEVEFSHEYWMRHALTLAKRARDEREVPVGAILVLNNRVIGEGWNRAIGLHDPTAHAEIMALRQGGLVMQNYRLIDATLYVTFEPCVMCAGAMIHSRIGRVVFGVRNSKRGAAGSLMNVLNYPGMNHCVEITEGILVDECAALLCDFYRMPRQVLNAQKKAQSSISSGGSSGGSSGSETPGASGSVIPRSSGGSSAGSTKDTITKTLKLRIVRPYNSAEVEKVVADEKNNREKIAMEKNKDKVKEACSKHLKVASYCTTQVERNACLFCKARKLDDKFYQKLRGQFPDAVFWQELGGIFRQLQKQAAEIYNQSLIELYYEIFIKGKGITNASRVEHYLSDVCYTRAAELFKNAAIASGLRSKVRSNFRLKELKNMKSGLPTTKSDNFPIPLVKQKGGQYTGFEISSHNSDFIIKIPFGRWQEKEEIDKYRPWEKFDFEQVRRSPKPISLLLSTQRRKRNRGWSKDEGTEAEIRKVMNGDYQTSYIEVKRGSKFGEKSAWMLNLSIDVPKIDKGVDPSIIGGIDVGVKSPLVCAINNAFSRYSISDNDLYRFNKKVFARRRILLKKNRHKRAGHGTKNKLKPITILTEKSGRFRKKLIERWACEIANFFIKNKVGTVQMENLESMKRKEDSYFNIRLRGFWPYAEMQNKIEFKLKQYGIKIRKVAPNNTSKTCSKCGHLNNYFSFEYRKKNKFPHFKCEKCNFKEDADYNAALNISNPKLKSTKEEP

SEQ ID NO: 130 - protein, 726 aa, synthetic construct
SEVEFSHEYWMRHALTLAKRARDEREVPVGAVLVLNNRVIGEGWNRAIGLHDPTAHAEIMALRQGGLVMQNYRLTDATLYVTFEPCVMCAGAMIHSRIGRVVFGVRNSKRGAAGSLINVLNYPGMNHCVEITEGILVDECAALLCDFYRMPRQVLNAQKKAQSSISSGGSSGGSSGSETPGASGSVTPKSSGGSSAGSTKDTITKTLKLRIVRPYNSAEVEKVVADEKNNREKIAIEKNKDMVKEACSKHLKVASYCTTQVERNACLFCKARKLDDKFYQKLRGQFPDAVFWQELGGIFRQLQKQAAEIYNQSLIELYYEIFIKGKGITNASRVEHYLSDVCYTRAAELFKNAAIASGLRSKVRSNFRLKELKNMKSGLPTTKSDNFPIPLVKQKGGQYTGFEISSHNDDFIIKIPFGRWQVKKEIDKYRPWEKFDFEQVRKSPKPISLLLSTQRRKRNKGWSKDEGTEAEIRKVMNGDYQTSYIEVKRGSKTGEKSAWMLNLSIDVPKIDKGVDPSIIGGIDVGVKSPLVCAINNSLSRYSISDNDLFHFNKKMFARRRILLKKNGHKRAGHGAKNKLKPITIMTEKSKRFRKKLIERWACEIADFFIKNKVGTVQMENLESMKRKEDSYFNVRLRGFWPYAEMQNKIEFKLKQYGIVVRKVAPNNTSKTCSKCGHLNNYFNFEYRKKNKFPHFKCEKCNFKENADYNAALNISNPKLKNTKGEP

SEQ ID NO: 131 - protein, 726 aa, synthetic construct
SEVEFSHEYWMRHALTLAKRARDGREVPVGAVLVLNNRIIGEGWNRAIGLHDPTAHAEIMALRQGGLATQNYRLIDATLYVTFEPCAMCAGAMVHSRIGRVVFGVRNSKRGAAGSLMNVLNYPGMDHRVEITGGILADECAALLCDFYRMPRRVFNAQKKAHSSINSGGSSGGSSGSVTPGTSESATPESSGGGFGGSAKNTITKTLQLRIVRPYNSAEVEKIVADEKNNREKIALEKNKDKVREACSKHLKVASYCTTQVERNACPFCKARKLDDKFYQKLWGQFPDAVFWQELGEILRQLQKQAAEIYNQSLIELYYEIFIKGRGFANASSVEHYLSDVCYTRAAGLFKNAAIASGLRGKVKSNFRLKELKNMKSGLPTTKSDNFPIPLVKQKGGQYTGFEISSHNDDFIIKIPFGRWQVKKEIDKYRPWEKFDFEQVRKSPKPISLLLSTQRRKRNKGWSKDEGTEAEIRKVMNGDYQTSYIEVKRGSKIGEKSAWMLNLSIDVPKIDKGVDPSIIGGIDVGVKSPLVCAINNVLSRYSISDNDLFHFNKKMFARRRILLKKNGHKRAGHGAKNKLKPITIMTEKSKRFRKKLIERWACEIADFFIKNKVGTVQMENLESMKRKEDSYFNIRLRGFWPYAEMQNKIEFKLKQYGIEIRKVAPNNTSKTCSKCGHLNDYFNFEYRKKNKFPHFKCEKCNFKENADYNAALNISNPKLKSTKEEP

SEQ ID NO: 132 - protein, 726 aa, synthetic construct
SEVEFSHEYWMRRALTLAKRARDEREVPVGAVLVLNNRVIGVGWNRAVGLHDPTAHAEIMALRQGGLVMQNHRLVDATLYVTFEPCVMCAGAMIHSRIGRVVFGVRNSKRGAAGSLTNVLNYPGMSHRVEITEGILADECAALLCDFYRMPRQVFNAQKKAQSNINPGGSSGGSSGSETPGTSESATPGSSGGSSGGSAKNTITKTLKLRIVRPYNSAEVEKIVADEKNNRERIALEKNKDKVKEACSKHLKMASYCTTQVERNACLFCKARKLDDKFYQKLRGQFPDAVFWQELGGIFRQLQKQAAEIYNQSLIELYYEIFIKGKGITNASRVEHYLSDVCYTRAAELFKNAAIASGLRSKVRSNFRLKELKNMKSGLPTTKSDNFPIPLVKQKGGQYTGFEISSHNSDFIIKIPFGRWQVKEEIDKYRPWEKFDFEQVRKSPKPISLLLSTQRRKKNKGWSKDEGTEAEIRRVMNGDYRTSYIEVKRGSKIGEKSAWMLNLSIDVPKIDKGVDPSIIGGIDVGVKSPLVCAINNSSSRYSICDNDLFRFNKKMFARRRILLKKNRLRRAGHGAKNKLKPITVLTKKSERFRKKLIERWVCEVADFFIKNKVGTVQMENLESMKRKEDSYFNIRLRGFWPYAEMQNKIEFKLKQYGIVVRKVAPNNTSKTCSKCGHLNNYFNFEYRKKNKFPHFKCEKCNFKEDADYNAALNISNPKLKSTKGEP

SEQ ID NO: 133 - protein, 726 aa, synthetic construct
SEVEFSHEYWMRHALTLAKRARDEREVPVGAVLVLNNRAIGEGWNRAIGLHDPTAHAEIMALRQGGLVMQNYRLTDATLYVTFEPCVMCAGAMIHSRIGRVVFGVRNNKHGAAGSLVNVLNYPGMNHRVEITEGILVDECAALLCDFYRMPRQVLNAQKKAQSSISSGGSSGGCSGSEMPGASESVTPKSSGGSSAGSTKNTITKTLKLRIVRPYNSAEVEKIVADEKNSREKIALEKNKDKVKEACSKHLKVAAYCTTQVERNACLFCKARKLDDKFYQKLRGQFPDAVFWQEISEIFRQLQKQAAVIYNQGLIELYYEIFIKGKGIANASRVEHYLSNVCYTRAAELFKNAAIASGLRNKIKSNFRLKELRNMKSGLPTTKSDNFPIPLVRQKGGQYTGFEISNHDGDFIIKIPFGRWRVKKEINKHRPWEKFDFEQVRKSPKPISLLLSTQRRKRNKGWSRDEGTEAEIRKVMNGDYQTSYIEVKRGSKIGEKSAWMLNLSIDVPKIDKGVDPSIIGGIDVGVKSPLVCAINNALSRYSISDNDLFHFNKKMFARRRILLRKNRHKRAGHGAKNKLKPITMMTEKSKRFRKKLIERWACEIADFFIKNKVGTVQMENLESMKRKEDSYFNIRLRGFWPYAEMQNKIEFKLKQYGIVVRKVAPNNTSKTCSKCGHLNNYFNFEYRKKNKFPHFKCEKCNFKEDADYNAALNISNPKLKSTKGEP

SEQ ID NO: 134 - protein, 726 aa, synthetic construct
SEVELSHEYWMRHALTLAKRARDEHEVPVGAVLVLNNRVIGEGWNRAIGLHDPTAHAEIMALRQGGLVMQNYRLTDATLYVTFEPCVMCAGAMIHSRIGRVVFGVRNSKRGAAGSLMNVLNYPGMNHCVEITEGILVDECAALLCDFYRMPRQVLNAQKKAQSSISSGGSSGGSSGSETSGASGSVTPKSSGGSSGGSAKNTITKTLKLRIVRPYNSAEVEKIVADEKNNREKIALERNKGKVREACSKHLKVASYCTTQVERNACPFCKARKLDDKFYQKLRGQFPDAVFWQELGEILRQLQKQAAEIYNQSLIELYYEIFIKGKGIASASRVGHYLSDVCYTRAAELFKNAAIASGLRGKVKSNFRLKELKNMRSGLPTTKSDNFPIPLVKQKGGQYTGFEINSHNDDFIIKIPFGRWQVKKEIDKYRPWEKFDFEQVRKSPKPISLLLSTQRRKRNKGWSKDEGTEAEIRKVMNGDYQTSYIEVKRGSKTGEKSAWMLNLSIDVPKIDKGVDPSIIGGIDVGVKSPLVCAINNAFSRYSISDNDLFRFNKKMFARRRILLKKNRHKRAGHGAKNKLKPISILTGKSERFRKKLIERWACEIADFFIKNKVGTVQMENLESMKRKEDSYFNIRLRGFWPYAEMQNKIEFKLKQYGIEIRKVAPNNTSKTCSKCGHLNNYFNFEYRKKNKFPHFKCEKCNFKENADYNAALNISNPKLMSTKEGP

SEQ ID NO: 135 - protein, 726 aa, synthetic construct
SEVEFSHEYWMRHALTLAKRARDEREVPVGAVLVLNNRVIGVGWNRAIGLHDPTAHAEIMALRQGGLVMQNYRLTDATLYVTFEPCVMCAGAMVHSRIGRVVFGVRNSKRGAAGSLMNVLNYPGMSHCVEITEGILVDECAALLCDFYHMPRQVLNAQKKAQSSISSGGSSGGSGGGETPGASESVTPKNSGGSSAGSTKNTITKTLKLRIVRPYNSAEVEKIVADEKNSREKIALEKNKDKVREACSKHLKVASYCTTQVERNACPFCKARKLDDKFYQKLRGQFPDAVFWQELGEILRQLQKQAAEIYNQSLIELYYEIFIKGRGFANASSVEHYLSDVCYTRAAELFKNAAIASGLRGKVKGNFRLKELKNMKSGLPTTKSDNFPIPLVKQKGGQYTGFEISSHNDDFIIKIPFGRWQVKKEIDKYRPWEKFDFEQVRKSPKPISLLLSTQRRKRNKGWSKDEGTEAEIRKVMNGDYQTSYIEVKRGSKIGEKSAWMLNLSIDVPKIDKGVDPSIIGGIDVGVRSPLVCAINNAFSRYSISDNDLFRFNKKMFARRRILLKKNRHKRAGHGAKNKLKPITILTEKSRRFRKKLIERWACEIANFFIKNKVGTVQMENLESMKRREDSYFNIRLRGFWPYAEMQSKIEFKLKQYGIKIRKVAPNNTSKTCSKCGHLNNYFNFEFRKKNKFPHFKCEKCNFKEDADYNAALNISNPKLKGTKEEP

SEQ ID NO: 136 - protein, 726 aa, synthetic construct
SEVEYSHEYWMRYALTLAKRARDEREVPVGAVLVLNNRVIGEGWNRAIGLHDPTAHAEIMALRQGGLVMQNYRLIDATLYVTFEPCVMCAGAMIHSRIGRVVFGVRNSKRGAAGSLMNVLNYPGMNHRVEITEGILADECAALLCDFYRMPRQVLNAQKRARSCISPGGSSGGSSGGETPGTSESATPESSGGSSGGSAKNTITKTLKLRIVRPYNSAEVEKIVADEKNNREKIALEKNKDKVKEACSKHLKVAAYCTTQVERSACLFCKARKLDDKFYQKLRGQFPDAVFWQELGGIFRQLQKQAAEIYNQSLIELYYEIFIKGKGITNASRVEHYLSDVCYTRAAELFKNAAIASGLRSKVRSNFRLKELKNMKSGLPTTKSDNFPIPLVKQKGGQYTGFEISSHNSDLIIKIPFGRWQVKEEIDKYRPWEKFDFEQVRKSPKPISLLLSTQRRKKNKGWSKDEGTEAEIRRVMNGDYQTSYIEVKRGSKIGEKSAWMLSLSIDVPKIDKGVDPSIIGGIDVGVKSPLVCAINNSFSRYSISDNDLFHFNKKMFARRRILLKKSKHKRAGHGAKNKLKPITILTEKSRRFRKKLIERWACEIADFFVKNKVGTVQMENLESMKRKEDSYFNIRLRGFWPYAEMQNKIEFKLKQYGIEIRKVAPNNTSKTCSKCGHLNNYFNFEYRKKNKFPHFKCEKCNFKENADYNAALNISNPKLKSTKEEP

SEQ ID NO: 137 - protein, 726 aa, synthetic construct
SEVEFSHEHWMRHALTLAKRARDEREVPVGAVLVLNNRVIGEGWNRAIGLHDPTAHAEIMALRQGGLVMQNYRLTDATLYVTFEPCVMCAGAMIHSRIGRVVFGVRNSKRGAAGSLMNVLNYPGMNHCVEITEGILVDECAALLCDFYRMPRQVLNAQKKAQSSISSGGSSGGSSGSETPGTSESATPESSSGGFGGSAKNTITKTLQLRIVRPYNSAEVEKIVADEKNNREKIALEKNKDKVKEACSKHLKVASYCTTQVERNACLFCKARKLDDKFYQKLRGQFPDAVFWQELGGIFRQLQKQAAEIYNQSLIELYYEIFIKGKGITNASRVEHYLSDVCYTRAAELFKNAAIASGLRGKVKSNFRLKELKNMKSGLPTTKSDNFPIPLVKQKGGQYAGFEISNHNGDFIIKIPFGRWQVKKEIDKYRPWEKFDFEQVRKSPKPISLLLSTQRRKRNKGWSKDEGTEAEIRKVMNGDYQTSYIEVKRGSKIGEKSAWMLNLSIDVPKIDKGVDPSIIGGIDVGVKSPLVCAINNAFSRYSISDNDLFHFNKKMFARRRILLKKNGHKRAGHGARNKLRPITVLTEKSKRFRKKLIERWACEIANFFIKNRVGTVQMENLESMKRKEDSYFNIRLRGFWPYAEMQNKIEFKLKQYGIKVRKVAPNNTSKTCSKCGHLNNYFSFEYRKKNKFPHFKCEKCNFKENADYNAALNISNPKLKSTKEEP

SEQ ID NO: 138 - protein, 726 aa, synthetic construct
SEVEFSHEYWMRHALTLAKRARDEREVPVGAVLVLNNRVIGEGWNRAIGLHDPTAHAEIMALRQGGLVMQNYRLTDATLYVTFEPCVMCAGAMIHSRIGRVVFGVRNSKRGAAGSLMNVLNYPGMNHCVEITEGILVDECAALLCDFYRMPRQVLNAQKKAQSSISSGGPSGGSSCSEMPGASESVTPKSSGGSSAGSTKNTITKTLKLRIVRPYNSAEVEKIVADEKNSREKIALEKNKDKVKEACSEHLKVAAYCTTQVERNACLFCKARKLDDKFYQELRGQFPDAVFWQEIGEIFRQLQKQAAEIYNQSLIELYYEIFIKGKGFANASSVEHYLSDVCYTRAAELFKNAAIASGLRGKVKSNFRLKELKNMRSGLPTTKSDNFPIPLVKQKGGQYAGFEISSHNDDFIIKIPFGRWQVKKEIDKYRPWEKFDFEQVRKSPKPISLLLSTRRRKRNKGWSKDEGTEAEIRKVMNGDYQTSYIEVKRGSKIGEKSAWMLNLSIDVPKIDKGVDPSIIGGIDVGVKSPLVCAINNAFGRCSISDNDLFHFNKKMFARRRILLKKNGHKRAGHGAKNKLKPITIMTEKSKRFRKKLIERWACEIADFFIKNKVGTVQMENLESMKRKEDSYFNIRLRGFWPYAEMQNKIEFKLKQYGIVVRKVAPNNTSKTCSQCGHLNNYFNFEYRKKNKFPYFKCEKCNFKENADYNAALNISNPQLKSTKGEP

SEQ ID NO: 139 - protein, 726 aa, synthetic construct
SEVEFSHEYWMRHALTLAKRARDEREVPVGAVLVLNNRVIGEGWNRAIGLHDPTAHAEIMALRQGGLVMQNYRLIDATLYVTFEPCVMCAGAMIHSRIGRVVFGVRNSKHGAAGSLVNVLNYPGMNHRVEITEGILADECAALLCDFYRMPRQVFGARRKAQSSISSGGSSGGSSCSETPGASESVTPKSSGGSSAGSTKNTITKTLKLRIVRPYNSAEVEKIVADEKNNREKIALEKNKDKVKEACSEHLKVAAYCTTQVERNACLFCKARKLDDRFYQKLRGQFPEAVFWQEIGEIFRQLQKQAAEIYNQSLIELYYEIFIKGKGFANASSVEHYLSDVCYTRAAELFKNAAIASGLRGKVKSNFRLKELKNMKSGLPTTKSDNFPIPLVKQKGGQYTGFEVSSHNDDFIIKIPFGRWQVKKEIDKYRPWEKFDFEQVRKSPRPISLLLSTQRRKRNKGWSKDEGTEAEIRKVMNGDYRTSYIEVKRGSKIGEKSAWMLNLSIDVPKIDKGVDPSIIGGIDVGVKSPLVCAINNAFSRYSISDNDLFHFNKKMFARRRILLKKSKHKRAGHGAKNKLKPITILTEKSKRFRKKLIERWACEIADFFIKNKVGTVQMENLESMKKKEDSYFNIRLRGFWPYAEMQNKIEFKLKQYGIEIRKVAPNNTSRTCSKCGHLNNYFNFEYRKKNKFPHFKCEKCNFKEDADYNAALNISNPRLKSTKEEP

SEQ ID NO: 140 - protein, 726 aa, synthetic construct
SEVEFSHEYWMRRALTLAKRARDEREVPVGAVLVLNNRVIGVGWNRAVGLHDPTAHAEIMALRQGGLVMQNYRLVEATLYVTFEPCIMCAGAMIHSRIGRVVFGVRNSKRGAAGSLMNVLNYPGMNHRVEITEGILADECAALLCDYYRMPRQVFNARKKAQSSINSGGSSGGSSGSETPGTSESATPKSSGGSPGGSAKNTITKTLKLRIVRPYNSAEVEKIVADEKNNREKIALEKNKDKVKEACSKHLKVAAYCTTQVERNACLFCKARKLDDKFYQKLRGQFPDAVFWQELGGIFRQLQKQAAEIYNQSLIELYYEIFIKGRGFANASSVEHYLSGVCYTRAAELFKNAAIASGLRGKVKGNFRLKELKNMKSGLPTTKSDNFPIPLVKQKGGQYTGFEISSHNDDFIIKIPFGRWQVKKEIDKYRPWEKFDFEQVRKSPKPISLLLSTQRRKRNKGWSKDEGTEAEIRKVMNGDYQTSYIEVKRGGRTGEKSAWMLNLSIDVPKIDKGVDPGIIGGIDVGVKSPLVCAINNASSRYSISDNDLFHFNKKMFARRRILLKKNRHKRAGHGAKNKLKPITIMTEKSKRFRKKLIERWACEIADFFIKNKVGTVQMENLESMKRKEDSYFNIRLRGFWPYAEMQNKIEFKLKQYGIEVRKVAPNNTSKTCSKCGHLNNYFNFEYRKKNKFPHFKCEKCNFKENADYNAALNISNPKLKSTKEEP

SEQ ID NO: 141 - protein, 726 aa, synthetic construct
SEVEFSHEYWMRHALTLAKRARDEREVPVGAILVLNNRVIGEGWNRAIGLHDPTAHAEIMALRQGGLVMQNYRLIDATLYVTFEPCVMCAGAMIHSRIGRVVFGVRNNKHGAAGSLVNVLDYPGMNHRVEITEGILADECAALLCDFYRMPRQVFNARKKAQSSISLGGSSGGSSGSETPGTSESATPESSGGSSGGSAKNTITKTLKLRIVRPYNSAEVEKIVADEKNYREKIALEKNKDKVKEACSEHLKVAAYCTTQVERNACLFCKARKLDDKFYQKLRGQFPGAVFWQEIGEIFRQLQKQAAEVYNQSLIELYYEIFIKGKGFANASSVEHYLSDVCYTRAAELFKNAAIASGLRGKVKSNFKLKELRSMRSGLPTTKSDNFPIPLVKQKGGQYTGFEISSHNDDFIIKIPFGRWQVKKEIDKYRPWEKFDFEQVRKSPKPISLLLSTQRRKKNKGWSKDEGTEAEIRRVMNGDYQTSYIEVKRGSKIGEKSAWMLNLSIDVPKIDKGVDPSIIGGIDVGVKSPLVCAINNAFSRYSISDNDLFHFNKKMFARRRILLKKSKHKRAGHGAKNKLKPITILTEKSKRFRKKLIERWACEIADFFIKNKVGTVQMENLESMKKKEDSYFNIRLRGFWPYAEMQNKIEFKLKQYGIEIRKVAPNNTSRTCSKCGHLNNYFNFEYRKKNKFPHFKCEKCNFKEDADYNAALNISNPKLKSTKEEP

SEQ ID NO: 142 - protein, 726 aa, synthetic construct
SEVEFSHEYWMRHALTLAKRARDEHEVPVGAILVLNNRVIGVGWNRAIGLHDPTAHAEIMALRQGGLVTQNYRLIDATLYVTFEPCVMCAGAMIHSRIGRVVFGVRNSKHGAAGSLVNVLNYPGMNHRVEITEGILADECAALLCDFYRMPRQVFNARKKAQSSINSGGSSGGSSGSETPGTSESATPKSSGGSSGGSAKNTITKTLKLRIVRPYNSAEVEKIVADEKNNREKIALEKNKGKVKEACSKHLEVAAYCTTQVERNACLFCKARKLDDKFYRKLRGQFPDAVFWQELGEIFRQLQKQAAEIYNQSLIELYYEIFIKGKGFANASSVEHYLSDVCYTRAAELFKNAAIASGLRGKVKSNFRLKELKNMKSGLPTTKSDNFPIPLVKQKGGQYTGFEINSHNDDFIIKIPFGRWQVRKEIDKYRPWEKFNFEQVRMSPKPISLLLSTQRRKRNKGWSKDEGTEAEIRKVMNGDYQTSYIEVKRGSKIGEKSAWMLNLSIDVPKIDKGVDPSIIGGIDVGVKSPLVCAINNAFSRYSISDNDLFRFNKKMFARRRILLGKNRHKRAGHGVKNKLKPITILTEKSGRFRKKLIERWACEIADFFVKNKVGTVQMENLESMKRKEDSYFNIRLRGFWPYAEMQNKIEFKLKQYGIKIRKVAPNNTSKTCSKCGHLNNYFSFEYRKKNKFPRFKCEKCNFKEDADYNAALNISNPKLKSTKEEP

SEQ ID NO: 143 - protein, 726 aa, synthetic construct
SEVEFSHEYWMRHALTLAKRARDEREVPVGAVLVLNNRVIGEGWNRAIGLHDPTAHAEIMALRQGGLVMQNYRLTDATLYVTFEPCVMCAGAMIHSRIGRVVFGVRNSKRGAAGSLMNVLNYPGMNHCVEITEGILVDECAALLCDFYRMPRQVLNAQKKAQSSISSGGSSGGSSVSETSGANESATPKSSGGSSAGSTKNTITKTLKLRIVRPYNSAEVEKIVADEKDNRERIALEKNKGKVKEACSKHLKVAAYCTTQVERNACLFCKARKLDDKFYQELRGQFPDAVFWQEIGEIFRQLQKQAAEIYNQSLIELYYEIFIKGKGFANAGSVEHYLSDVCYTRAAELFKNAAIASGLRGKVKSNFRLKELKNMKSGLPTTKSDNFPIPLVKQKGGQYTGFEISSHNDDFIIKIPFGRWQVRKEIDKYRPWEKFDFEQVRKSPKPISLLLSTQRRKRNKGWSKDEGTEAEIRKVMNGDYQTSYIEVKRGSKTGEKSAWMLNLSIDVPKIDKGVDPSIIGGIDVGVKSPLVCAINNSLSRYSICDNDLFRFNKKMFARRRILLKKNRHKRAGHGAKNKLKPITILTKKSERFRKKLIERWACEVADFFIKNKVGTVQMENLESMKRKEDSYFNIRLRGFWPYAEMQDRIEFKLKQYGIEIRRVAPANTSRTCSKCGHLNNYFNFEYRKENKFPHFKCEKCNFREDADYNAALNISSPKLKSTKEEP

SEQ ID NO: 144 - protein, 726 aa, synthetic construct
SEVEFSHEYWMRHALALAKRARDEREVPVGAILVLNNRVIGEGWNRAIGLHDPTAHAEIMALRQGGLVMQNYRLIDATLYVTFEPCVMCAGAMIHSRIGRVVFGVRNNKHGAAGSLVNVLNYPGMNHRVEITEGILADECAALLCDFYRMPRQVFNARKKAQSSINPGGSSGGSGGSETPGTSESPTPESSRGSPGGSAKNTITKTLKLRIVRPYNSAEVEKIVAEEKDNREKIALEKNKDKVREACGKHLKMASYCTTQVERNACLFCKARKLDDKFYQKLRGQFPDAVFWQEIGEIFRQLQKQAAEVYNQSLVELYYEILIKGKGIANASSVEHYLSDVCYTRAAELFKNAAIASGLRNKIKSNFRLKELRNMRSGLPTTKSDNFPIPLVRQKGGQYTGFEISNHDGDFIIKIPFGRWQVKKEINKHRPWEKFDFEQVRKSPKPISLLLSTQRRKRNKGWSKDEGTEAEIRKVMNGDYQTSYIEVKRGSKTGEKSAWMLNLSIDVPKIDKGVDPSIIGGIDVGVKSPLVCAINNAFSRYSISDNDLFRFNKKMFARRRILLKKNRHKRAGHGAKNKLKPISILTGKSERFRKKLIERWACEIADFFIKNKVGTVQMENLESMKRKEDSYFNIRLRGFWPYAEMQNKIEFKLKQYGIVVRKVAPNNTSKTCSKCGHLNNYFNFEYRKKNKFPHFKCEKCNFKEDADYNAALNISNPKLKSTKGEP

SEQ ID NO: 145 - protein, 726 aa, synthetic construct
SEVEFSHEYWMRHALTLAKRARDEREVPVGAILVLNNRVIGEGWNRAIGLHDPTAHAEIMALRQGGLVMQNYRLIDATLYVTFEPCVMCAGAMVHSRIGRVVFGVRNSKRGAAGSLMNVLDYPGMDHRVEITEGILADECAALLCDFYRMPRQVLNAQRKAQSSISPGGSSGGSSGSETPGASESVTPKSSGGSSGGSAKNTITKTLKLRIVRPYNSAEVEKIVADEKNNREKIALEKNKDKVREACSKHLKVASYCTTQVERNACPFCKARKLDDKFYQKLRGQFPDAVFWQELGEILRQLQKQAAEIYNQSLIELYYEIFIKGRGFANASSVEHYLSGVCYTRAAELFKNAAIASGLRGKVKSNFRLKELKNMKSGLPTTKSDNFPIPLVKQKGGQYTGFEISSHNDDFIIKIPFGRWQVKEEIDKYRPWEKFDFEQVRKNPKPISLLLSTQRRKRNKGWSKDEGTEAEIRKVMNGDYQTSYIEVKRGSKIGEKSAWMLNLSIDVPKIDKGVDPSIIGGIDVGVKSPLVCAINNAFSRYSISDNDLFRFNKKVFARRRILLKKNRHKRAGHGVKNKLKPITILAEKSKRFRKKLIERWACEIADFFVKNKVGTVQMENLESMKRREDSYFNIRLRGFWPYAKMLNRIEFKLKQYGIKIRKVAPNNTSKTCSKCGHLNNYFNFEYRKKNKFPHFKCEKCNFKENADYNAALNISNPKLKSTKEEP

SEQ ID NO: 146 - protein, 726 aa, synthetic construct
SEVEFSHEYWMRHALALAKRARDEREVPVGAVLVLNNRVIGEGWNRAIGLHDPTAHAEIMALRQGGLVMQNYRLTDATLYVTFEPCVMCAGAMIHSRIGRVVFGVRNSKRGAAGSLMNVLNYPGMNHCVEITEGILVDECAALLCDFYRMPRQVLNAQKKAQSSISSGGSSGGSSGSETPGASESVTPKSSVGSSAGSTKNTITKTLKLRIVRPYNSAEVEKIVADEKDNRERIALEKNKDKVKEACSEHLKVAAYCTTQVERSACLFCKARKLDDKFYQKLRGQFPDAVFWQEIGEIFRQLQKQAAEIYNQSLIELYYEIFIKGKGIANASSVEHYLSDVCYTRAAELFKNAAIASGLRNKVKSNFRLKELRSMKSGLPTTKSDNFPIPLVKQKGGQYTGFEISSHNDDFIIKIPFGRWQEKKEINKYRPWEKFDFEQVRKSPKPISLLLSTQRRKRNKGWSKDEGTEAEIRKVMNGNYQTSYIEVKRGSKIGEKSAWMVNLSIDVPKIDKGVDPSIIGGIDVGVKSPLVCAVNNALSRYSIDDNDLFHFNKKMFARRRILLKKSRHKRAGHGAKNKLKPITILTEKSRRFRKKLIERWACEIADFFIKNKVGTVQIENLESMKRKEDSYFNIRLRGFWPYAEMQNKIEFKLKQYGIEVRKVAPNNTSKTCSKCGHLNDYFSFEYRKKNKFPHFKCEECNFKENADYNAALNISNSKLTSTKEEP

SEQ ID NO: 147 - protein, 726 aa, synthetic construct
SEVEFSHEYWMRHALTLAKRARDEREVPVGAVLVLNNRAIGVGWNRAIGLHDPTAHAEIMALRQGGLVMQNYRLIDATLYVTFEPCVMCAGAMVHSRIGRVVFGVRNSKRGAAGSLMNVLDYPGMGHRVEITEGVLADECAALLCDFYCMPRQVFNAQKRAQSSINSDGSSGGSSGSETPGTSESATPESSGGGSSGSAKNTITKTLQLRIVRPYNSAEVEKIVADEKNNREKIALEKNKDKVREACSKHLKVASYCTTQVERNACPFCKARKLDDKFYQKLKGQFPDAVFWQELGGILRQLQKQAAEIYNQSLIELYYEIFIKGRGFANASSVEHYLSDVCYTRAAELFKNAAIASGLRGKIKSNFRLKELKNMKSGLPTTKSDNFPIPLVKQKGGQYTGFEISNHNGDFIIKIPFGRWQVKKEINKFRPWEKFDFEQVRKSPKPISLLLSTQRRKRNKGWSKDEGTEAEIRKVMNGDYQISYIEVKRGSKIGEKSAWTLNLSVDVPKIDKGVDPSIIGGIDVGVKSPLVCAINNALSRYSISDNDLFHFNKKVFARRRILLKKNRHRRAGHGAKNKLKPITILTEKSKRFRKKLIERWACEIADFFIKNKVGIVQMENLESMKRREDSYFNIRLRGFWPYAEMQNKIEFKLKQYGIEVRKVAPNNTSKTCSKCGHLNNYFNFEYRKKNKFPHFKCEKCNFKENADYNAALNISNPKLKSTKEEP

SEQ ID NO: 148 - protein, 726 aa, synthetic construct
SEVEFSHEYWMRHALTLAKRARDEREVPVGAILVLNNRVIGEGWNRAIGLHDPTAHAEIMALRQGGLVMQNYRLIDATLYVTFEPCVMCAGAMIHSRIGRVVFGVRNSKRGAAGSLMNVLNYPGMNHRVEITEGILADECAALLCDYYRMPRQVFNARKKAQSSINSGGSSDGGSGSETPGTSESATPESSGGSSGGSAKNTITKTLKLRIVRPYNSAEVEKIVADEKSNREKIALEKNKDKVKEACSEHLKVASYCTTQVERNACLFCKARKLDDKFYQKLRGQFPDAVFWQELGEILRQLQKQAAEIYNQSLIELYYEIFIKGRGFANASSVEHYLSDVCYTRAAELFKNAAIASGLRGKVKSNFRLKELKNMKSGLPTTKSDNFPIPLVKQKGGQYTGFEISSHNDDFIIKIPFGRWQVKKEIDKYRPWEKFDFEQVRKSPKPISLLLSTQRRKRNKGWSKDEGTEAEIRKVMNGDYQTSYIEVKRGSKIGEKSAWMLSLSIDVPKIDKGVDPSIIGGIDVGVKSPLVCAINNAFSRYSISDNDLFRFNKKMFARRRILLKKNRHKRAGHGAKNKLKPISILTGKSERFRKKLIERWACEIADFFIKNKVGTVQMENLESMKRKEDSYFNTRLRGFWPYAEMQNKIEFKLKQYGIEIRKVAPNNTSKTCSKCGHLNNYFNFEYRKKNKFPHFKCEKCNFKENADYNAALNISNPKLKSTKEEP

SEQ ID NO: 149 - protein, 726 aa, synthetic construct
SEVEFSHEYWMRHALTLAKRARDEREVPVGAVLVLNNRVIGEGWNRAIGLHDPTAHAEIMALRQGGLVLQNYRLADATLYVTFEPCVLCAGAMVHSRIGRVVFGARNSKRGAAGSLMNILNYPGMNHRVEITEGILADECAALLCDFYRMPRQVFSARKKAQSSINSGGSSGGNSGSKTPSTSESATPESSGGSSGGSAKNTITKTLKLRIVRPYNSAEVEKIVADEKNNREKIALEKNKDKVKEACSKHLKVAAYCTTQVERNACQFCKARKLDDKFYQKLRGQFPDAVFWQEIGEIFRQLQKQAAEIYNQSLIELYYEIFIKGKGFANASSVEHYLSDVCYSRAAELFKNAAIASGLRGKVKSNFRLKELKNMKSGLPTTKSDNFPIPLVKQKGGQYTGFEISSRNDDFIIKIPFGRWQVKKEIDKYRPWEKFDFEQVRKSPKPISLLLSTQRRKRNKGWSKDEGTEAEIRKVMNGDYQTSYIEVKRGSKTGEKSAWMLNLSIDVPKIDKGVDPSIIGGIDVGVKSPLVCAINNAFSRYSISDNDLFRFNKKMFARRRILLGKNRHKRAGHGVKNKLKPITILTEKSGRFRKKLIERWACEIADFFVKNKVGTVQMENLESMKRKEDSYFNIRLRGFWPYAEMQNKIEFKLKQYGIKVRKVAPNNTSKTCSKCGHLNNYFSFEYRKKNKFPHFKCEKCNFKGNADYNAALNISNPKLKSTKEEP

SEQ ID NO: 150 - protein, 726 aa, synthetic construct
SEVEFSHEYWMRHALTLAKRARDEREVPVGAVLVLNNRVIGEGWNRAIGLHDPTAHAEIMALRQGGLVMQNYRLTDATLYVTFEPCVMCAGAMIHSRIGRVVFGVRNSKRGAAGSLMNVLNYPGMNHCVEITEGILVDECAALLCDFYRMPRQVLNAQKKAQPSISSGGSSGGSSGSETPGASESVTPKSSGGGSAGSTKNTITKTLKLRIVRPYNSAEVERIVADEKNSREKTALEKNKDKVKEACSEHLKVAAYCTTQVERNACLFCKARKLDDRFYQKLRGQFPDAVFWQEIGEIFRQLQKQSAEIYNQSLIELYYEIFIKGKGFANASSVEHYLSDVCYTRAAELFKNAAIASGLRGKVKSNFRLKELKNMKSGLPTTKSDNFPIPLVKQKGGQYTGFEISNHNDDFIIKIPFGRWQVKKEIDKYRPWEKFDFEQVRKSPKPISLLLSTQRRKRNKGWSKDEGTEAEIRKVMNGDYQTSYIEVKRGSKIGEKSAWMLNLSIDVPKIDKGVDPSIIGGIDVGVKSPLVCAINNALSRYSISDNDLFHFNKKMFARRRILLKKNRHRRAGHGAKNKLKPITILTEKSGRFRKKLIERWACEIANFFIKNKVGTVQMENLESMKRKEDSYFNIRLRGFWPYAEMQNKIEFKLKQYGIKIRKVAPNNTSKTCSKCGHLNNYFSFEYRKKNKFPHFKCEKCNFKEDADYNAALNISNPKLKSTKEEP

SEQ ID NO: 151 - protein, 726 aa, synthetic construct
SEVEFSHEYWMRHALTLAKRARDEGEVPVGAVLVLNNRVIGEGWNRAIGLHDPTAHAEIMALRQGGLVMQNYRLVDATLYVTFEPCVLCAGAMVHSRIGRVVFGVRNSKRGAAGSLMNVLNYPGMNHRVEITEGILADECAALLCDFYRMPRQVFNAQKKARSNINSGSSSGGSSGSETPGTSESATPVSSSGSSGGSAKNTITKTLKLRIVRPYNSAEVEKIVADEKNNREKIALAKNKDKVKEACSEHLKVAAYCTTQVERNACLFCKARKLDDKFYQKLRGQFPDAVFWQEIGEIFRQLQKQAAEIYNQSLVELYYEIFIKGKGFANASSVEHYLSDVCYTRAAELFKNAAIASGLRGKVKSNFRLKELKNMKSGLPTTKSDNFPIPLVKQKGGQYTGFEISSHNDDFIIKIPFGRWQVKGEIDKYRPWEKFDFEQVRKNPKPISLLLSTQRRKGNKGWSKDEGTEAEIRKVMNGDYQTSYIEVKRGSKIGEKSAWMLNLSIDVPQIDKGVDPSIIGGIDVGVKSPLVCAINNAFSRYSISDNDLYRFNKKMFARRRILLKKSKHKRAGHGAKNKLKPITILTEKSGRFRKKLIERWACEIADFFIKNKVGTVQMENLEGMKRKEDSYFNIRLRGFWPYAEMQNKIEFKLKQYGIEIRKVAPNNTSKTCSKCGHLNNYFNFEYRKKNKFPHFKCEKCNFKENADYNAALNISNPKLKSTKEEP

SEQ ID NO: 152 - protein, 726 aa, synthetic construct
SEVEFSHEYWMRHALTLAKRARDEREVPVGAILVLNNRVIGEGWNRAIGLHDPTAHAEIMALRQGGLVMQNYRLIDATLYVTFEPCVMCAGAMIHSRIGRVVFGVRNSKHGAAGSLVNVLNYPGMNHRVEITEGVLADECAALLCDFYRMPRQVFGARRKAQSSINPGGSSGGSSGSETPGTSESPTPESPGGSSGGSAKNTITKTLKLRIVRPYNSAEVEKIVADEKNNREKIALEKNKDKVREACSKHLKMASYCTTQVERNACLFCKARKLDDKFYQKLRGQFPDAVFWQELGGIFRQLQRQAAEIYNQSLIELYYEIFIKGKGITNASRVEHYLSDVCYTRAAELFKNAAIASGLRSKVRSNFRLKELKNMKSGLPTTKSDNFPIPLVKQKGGQYTGFEISSHNSDFIIKIPFGRWQVKEEIDKFRPWEKFDFEQVRKSPKPISLLLSTQRRKKNKGWGKDEGTEAEIRKVMSGDYQTSYIEVKRGSKTGEKSAWMLNLSIDVPKIDKGVDPSIIGGIDVGVKSPLVCAVNNAFSRYSIGDNDLFHYNKKMFARRRILLKKNRHKRAGHGAKNKLKPISILTEKSKRFRKKLIERWACEIADFFIKNKVGTVQMENLESMKRKEDSYFNIRLRGFWPYAEMQNKIEFKLKQYGIKVRKVAPNNTSKTCSKCGHLNNYFSFEYRKKNKFPHFKCEKCNFKENADYNAALNISNPKLKSTKEEP

SEQ ID NO: 153 - protein, 726 aa, synthetic construct
SEVEFSHEYWMRYALTLAKRARDEREVPVGAVLVLNNRVIGEGWNRAIGLHDPTAHAEIMALRQGGLVMQNYRLSDATLYVTFEPCVMCAGAMIHSRIGRVVFGVRNSKRGAAGSLMNVLNYPGMNHCVEITEGILVDECAALLCDFYRMPRQVLNAQKKAQSSISPGGSSGGCSGSEMPGASESVTPKSSGGSSAGSTKNTITKTLKLRIVRPYNSAEVEKIVADEKNSREKIALERNKDKVKEACSEHLKVAAYCTTQVERNACLFCKARKLDDKFYQKLRGQFPDAVFWQELGEILRQLQKQAAEIYNQSLIELYYEIFIKGRGFANASSVEHYLSGVCYTRAAELFKNAAIASGLRGKVKSNFRLKELKNMKSGLPTTKSDNFPIPLVKQKGGQYTGFEISSHNSDFIIKIPFGRWQVKEEIDKYRPWEKFDFEQVRKNPKPISLLLSTQRRKRNKGWSKDEGTEAEIRKVMNGDYQTSYIEVKRGSKIGEKSAWMLNLSIDVPKIDKGVDPSIIGGIDVGVKSPLVCAINNAFSRYSISDNDLFRFNKKVFARRRILLKKNRHKRAGHGTKNKLKPITTLTEKSGRFRKKLIERWACEIADFFIKNKVGTVQMENLESMKRKEDSYFNIRLRGFWPYAEMQNKIEFKLKQYGIEIRRVAPNNTSRTCSKCGHLNNYFDFEYRRKYKFPHFKCEKCNFKEDADYNAALNISNPKLKSTKEEP

SEQ ID NO: 154 - protein, 726 aa, synthetic construct
SEVEFSHEYWMRHALTLAKRARDEREVPVGAVLVLNNRVIGEGWNRAIGLHDPAAHAEIMALRQGGLVMQNYRLIGATLYVTFEPCVMCAGAMIHSRIGRVVFGVRNSKRGAAGSLMNVLNHPGMNHCVEITEGILVDECAALLCDFYRMPRQVLNAQKKAQSSISPGGSSGGSSGSETPGASESVTLKNSGGSSGGSAKNTITKTLKLRIVRPYNSAEVEKIVADEKNNREKIALEKNKDKVKEACSKHLEVAAYCTTQVERNACLFCKARKLDDKFYQKLRDQFPDAVFWQELGEIFRQLQKQAAEIYNQSLIELYYEIFIKGKGFANASSVEHYLSDVCYTRAAELFKNAAIASGLRGKVKSNFRLKELKNMKSGLPTTKSDNFPIPLVKQKGGQYTGFEISSHNDDFIIKIPFGRWQVKEEIDKYRPWEKFDFEQVRKNPKPISLLLSTQRRKGNKGWSKDEGTEAEIRKVMNGDYQTSYIEVKRGSKIGEKSAWMLNLSIDVPKVDKGVDPSIIGGIDVGVKSPLVCAINNAFSRYSISDNDLFRFNKKVFARRRILLKKNRHKRAGHGTKNKLKPITILTEKSGRFRKKLIERWACEIANFFIKNKVGTVQMEYLEGMKRKEDSYFNIRLRGFWPYAEMQNKIEFKLKQYGIKIRKVAPNNTSKTCSKCGHLNNYFSFEYRRKNKFPHFKCEKCNFKENADYNAALNISNPKLKSTKEEP

SEQ ID NO: 155 - protein, 726 aa, synthetic construct
SEVEFSHEYWMRHALTLAKRARDEREVPVGAVLVLNNRVIGEGWNRAIGLNDPTVHAEIMALRQGGLVMQNHRLIDATLYVTFEPCVMCAGAMIHSRIGRVVFGVRNSKRGAAGSLMNVLNCPGMNHRVEVTEGILADECAALLCDFYRMPRQVFNAQKKARSNINSGGSSGGSSGSETPGTSESASPESSGGSSGGSAKNTITKTLKLRIVRPYNSAEVEKIVADEKNNREKVALEKNKDKVREACSEHLKVAAYCTTQVERNACLFCKARKLDDKFYQKLRGQFPDAVFWQEIGEIFRQLQKQAAEIYNQSLIELYYEIFIKGKGFANASSVEHYLSDVCYTRAAELFKNAAIASGLRGKVKSNFRLKELKNMKSGLPTTKSDNFPIPLVKQKGGQYTGFEVSSHNDDFIIKIPFGRWQVKKEIDKYRPWEKFDFEQVRKSPKPISLLLSTQRRKRNKGWSKDEGTGAEIRKVMNGDYQTSYIEVKRGSKTGEKSAWMLNLSIDVPKIDKGVDPSIIGGIDVGVKSPLVCAINNAFSRYSISDNDLFRFNKKMFARRRILLKKNRHKRAGHGAKNKLKPITILTEKSKRFRRKLIERWACEIADFFIKNKVGTVQMENLESMKRKEDSYFNIRLRGFWPYAEMQDKIEFKLKQYGIEIRKVAPNNTSKTCSRCGHLNNYFNFEYRRKNKFPHFKCEKCSFKENADYNAALNISNPKLKSTKEEP

SEQ ID NO: 156 - protein, 726 aa, synthetic construct
SGVEFSHEYWMRHALTLAKRARDEREVPVGAVLVLNNRVIGEGWNRAIGLHDPTAHAEIMALRQGGLVMQNYRLTDATLYVTFEPCVMCAGAMIHSRIGRVVFGVRNSKRGAAGSLMNVLNYPDMNHCVEITEGILVDECAALLCDFYRMPRQVLNAQKKVQSSISSGGSSGGSSGSETPGASESATPKSSGGSSASSTKNTITKTLKLRVVRPYNSAEVEKIVADEKNNRERIALEKNKDKVKEACSKHLKVAAYCTTQVERNACLFCKARKLDDKFYQKLRDQFPDAVFWQEIGEIFRQLQRQAAEIYNQSLIELYYEIFIKGKGFANASSVEHYLSDVCYARAAELFKNAAIASGLRGKVKSNFRLKELKNMKSGLPTTKSDNFPIPLVKQKGGQYAGFEISSHNDDFIIKIPFGRWQVKKEIDKYRPWEKFDFEQVRKSPKPISLLLSTQRRRRNKGWSKDEGTEAEIRKVMNGDYQTSYIEVKRGSKIGEKSAWMLNLSIDVPKIDKGVDPSIIGGIDVGVKSPLVCAINNAFSRYSISDNDLFRFNKKMFARRRILLGKNRHKRAGHGVKNKLKPITIMTEKSKRFRKKLIERWACEIADFFIKNKVGTVQMENLESMKRREDSYFNIRLRGFWPYAEMQNKIEFKLKQYGIKVRKVAPNNTSKTCSRCGHLNNYFSFEYRRKNKFPHFKCEKCNFKENADYNAALNISNPKLKSTKEEP

SEQ ID NO: 157 - protein, 726 aa, synthetic construct
SEVEFSHEYWMRHALTLAKRARDEHEVPVGAVLVLNNRAIGEGWNRAIGLHDPTAHAEIMALRQGGLVMQNYRLTDATLYVTFEPCVMCAGAMIHSRIGRVVFGVRNSKRGAAGSLMNVLNYPGMNHCVEITEGILVDECAALLCDFYRMPRQVLNAQKKAQSSISSGGSSGGSSGSETPGASGSVIPRSSGGSSAGSTKDTITKTLKLRIVRPYNSAEVEKVVADEKNNREKIAMEKNKDKVKEACSKHLKVASYCTTQVERSACLFCKARKLDDKFYQKLRGQFPDAVFWQELGGIFRQLQKQAAEIYNQSLIELYYEIFIKGKGITNASRVEHYLSDVCYTRAAELFKNAAIASGLRSKVRSNFRLKELKNMKSGLPTTKSDNFPVPLVKQKGGQYTGFEISSHNDDFIIKIPFGRWQVKKEIDKYRPWEKFDFEQVRKSPKPISLLLSTQRRKRNKGWSKDEGTEAEIRKVMNGDYQISYIEVKRGSKIGEKSAWMLNLSVDVPKIDKGVDPSIIGGIDVGVKSPLVCAINNALSRYSISDNDLFHFNKKMFARRRILLKKNRHRRTGHGARNKLKPITVLTEKSERFRKKLIERWACEIANFFIKNKVGTVQMENLESMKRREDSYFNIRLRGFWPYAEMQNKIEFKLKQYGIEIRKVAPNNTSKTCSKCGHLNNYFNFEYRKKNKFPHFKCEKCNFKENADYNAALNISNPRLKSTKEEP

SEQ ID NO: 158 - protein, 726 aa, synthetic construct
SEVEFGHEYWMRHALTLAKRARDEREVPVGAVLVLNNRVIGEGWNRAIGLHDPTAHAEIMALRQGGLVMQNHRLVDATLYVTFEPCVLCAGAMVHSRIGRVVFGVRNSKRGAAGSLMNVLNYPGMNHRVEITEGILADECAALLCDFYRMPRQVFNARKKARSNINSGGSSGGSSGSETPGTSESATPKSSGGSSGGSAKNTITKTLKLRIVRPYNSAEVEKIVADEKNNREKIALEKNKDKVKEACSKHLKVASYCTTQVERNACLFCKARKLDDKFYQKLRGQFPDAVFWQELGEIFRQLQKQAAEIYNQSLIELYYVIFIKGKGLANASSVEHYLSDVCYTRAAELFKNAAIASGLRGKVKSNFKLKELKNMKSGLPTTKSDNFPIPLVKQKGGQYTGFEISSHNSDFIIKIPFGRWQVKEEIDKYRPWEKFDFEQVRKSPKPISLLLSTQRRKKNKGWSKDEGTEAEIRRVMNGDYQTSYIEVKRGSKIGEKSAWMLNLSIDVPKIDKGVNPSIIGGIDVGVKSPLVCAINNSSSRYSICDNDLFRFNKKMFARRRILLKKNRHKRAGHGAKNKLKPITILTERSKRFRKKLIERWACEIADFFIKNKVGTVQMENLESMKRKEDSYFNIRLRGFWPYAEMQNKIEFKLKQYGIEIRKVAPNNTSRTCSKCGHLNNYFNFEYRKENKFPHFKCEKCNFKEDADYNAALNISNPKLKSTKEEP

SEQ ID NO: 159 - protein, 726 aa, synthetic construct
SEVEFSHEYWMRHALTLAKRARDEREVPVGAVLVLNNRVIGEGWNRAIGLHDPTAHAEIMALRQGGLVMQNYRLVDATLYVTFEPCVLCAGAMVHSRIGRVVFGVRNSKRGAAGSLMNVLNHPGMNHRVEITEGILADECAALLCDFYRMPRQVFNAQKKARSNINSGGSSGGSSGSETPGTSESATPVSSSGSSGGSAKNTITKTLKLRIVRPYNSAEVEKIVADEKNNREKIALEKNKDKVKEACSEHLKVAAYCTTQVERNACLFCKARKLDDKFYQKLRGQFPDAVFWQEIGEIFRQLQKQAAEIYNQSLIELYYEIFIKGKGFANASSVEHYLSDVCYTRAAELFKNAAIASGLRGKVKSNFRLKELKNMKSGLPTTKSDNFPIPLVKQKGGQYTGFEISSHNDDFIIKIPFGRWQMKKEVDKYRPWEKFDFEQVRKSPKPISLLLSTQRRKRRKGWSKDEGTEAEIRKVMNGDYQTSYVEVKRGSKIGEKSAWMLNLSIDVPKIDKGVDPSIVGGIDVGVKSPLVCAIDNALSRYSISDNDLFHFNKKMFARRRILLKKNRHRRAGHGAKNKLKPISILSEKSERFRKKLIERWACEIADFFIKNKVGTVQMENLESMKRREDSYFNIRLRGFWPYAKMLNKIEFKLKQYGIEIRKVAPNNTSKTCSKCGHLNNYFNFEYRKKNKFPHFKCEKCNFKENADYNAALNISNPKLKSTKGEP

SEQ ID NO: 160 - protein, 726 aa, synthetic construct
SEVEFSHEYWMRHALTLAKRARDEREVPVGAILVLNNRVIGEGWNRAIGLHDPTAHAEIMALRQGGLVMQNYRLIDATLYVTFEPCVMCAGAMIHSRIGRVVFGVRNSKHGAAGSLVNVLNYPGMNHRVEITEGILADECAALLCDFYRMPRQVFNARKKAQSSINPSGSSGGSSGSVTPGTSESATPESSGGGFGGSAKNTITKTLQLRIVRPYNSAEVEKIVADEKNNREKIALEKNKDKVKEACSKHLKVASYCTTQVERNACLFCKARKLDDKFYQKLRGQFPDAVFWQELGEIFRQLQKQAAEIYNQSLIELYYEIFIKGKGLANASSVEHYLSDVCYTRAAELFKNAAIASGLRGKVKSNFRLKELKNMKSGLPTTKSDNFPVPLVKQKGGQYTGFEISSHNDDFIIKIPFGRWQVKKEIDKYRPWEKFDFEQVRKSPKPISLLLSTQRRKRNKGWSKDEGTEAEIRKVMNGDYQTSYIEVKRGSKIGEKSAWMLNLSIDVPKIDKGVDPSIIGGIDVGVKSPLVCAINNAFSRYSISDNDLFRFNKKMFARRRILLGKNRHKRAGHGVKNKLKPITILTEKSGRFRKKLIERWACEIADFFVKNKVGTVQMENLESMKRKEDSYFNIRLRGFWPYAEMQNKIEFKLKQYGIEIRKVAPNNTSKTCSKCGHLNNYFNFEYRKMNKFPHFKCEKCNFKENADYNAALNISNPKLKSTKEEP

SEQ ID NO: 161 - protein, 726 aa, synthetic construct
SEVEFSHEYWMRHALTLAKRARDEREVPVGAVLVLDNRVIGEGWNRAIGLHDPTAHAEIMALRQGGLVMQNYRLSDATLYVTFEPCVMCAGAMIHSRIGRVVFGVRNSKRGAAGSLMNVLNYPGMNHCVEITEGILVDECAALLCDFYRMPRQVLSAQKKAQSSVSSGGSSGGSSGSETPGASGSVTPKSSVGGSAGSTKNTVTKTLKLRIVRPYNSAEVEKIVADEKNNREKVALEKNKDKVKEACSEHLKVAAYCTAQVERNACLFCKARKLDDKFYQKLKGQFPDAVFWQEIGEIFRQLQKQAAEIYNQSLIELYYEIFIKGKGFANASSVEHYLSDVCYTRAAELFKNAAIASGLRGKVKSNFRLKELKNMKSGLPTTKSDNFPIPLVKQKGGQYTGFEISSHNDDFIIKIPFGRWQVKKEIDKYRPWEKFDFEQVRKSPKPISLLLSTQRRKRNKGWSKDVGTEAEIRKVMNGDYQTSYIEVKRGSKIGEKSAWMLNLSIDVPKIDKGVDPSIIGGIDVGVKSPLVCAINNAFSRYSISDNDLFRFNKKMFARRRILLKKNRHQRAGHGAKNKLKPITILTEKSGRFRKKLIERWACEIADFFIKNKVGTVQMENLESMKRKEDSYFNIRLRGFWPYAEMQNKIEFKLKQYGIKIRKVAPNNTSKTCSKCGHLNNYFSFEYRKKNKFPHFKCEKCNFKENADYNAALNISNPKLMSTKEEP

SEQ ID NO: 162 - protein, 726 aa, synthetic construct
SEVEFSHEYWMRHALSLAKRARDEREVPVGAVLVLNNRVIGEGWNRAIGLHDPTAHAEIMALRQGGLVMQNYRLIDATLYVTFEPCVMCAGAMIHSRIGRVVFGVRNNKRGAAGSLMNVLNYPGMNHRVEITEGILADECAALLCDFYCMPRQVLNAQKKARSCINSGGSSGGSSGSETPGTSESATPESSGGSSGGSAKNTITKTLKLRIVRPYNSAEVEKIVADEKNNREKTALEKNKDKVKEACSKHLKVAAYCTTQVERNACLFCKARKLDDKFYQKLRGQFPDAVFWQEIGEIFRQLQKQAAEIYNQSLIELYYEIFIKGKGFANASSVEHYLSDVCYTRAAELFKNAAIASGLRGKVKSNFRLKELKNMKSGLPTTKSDNFPIPLVKQKGGQYTGFEISSHNDDFIIKIPFGRWQVKKEIDKYRPWEKFDFEQVRKSPKPISLLLSTQRRKRNKGWSKDEGTEAEIRRVMNGDYQTSYIEVKRGSKIGEKSAWMLNLSIDVPKIDKGVDPSIIGGIDVGVRSPLVCAINNAFSRYSISDNDLFRFNKKMFARRRILLKKNRHKRAGHGAKNKLRPITILTEKSRRFRKKLIERWACEIADFFIKNKVGTVQMESLESMKRKEDSYFNIRLRGFWPYAEMQNKIEFKLKQYGIKIRKVAPNNTSKTCSMCGHLNNYFNFEYRKRNKFPHFKCEKCNYKEDADYNAALNISNPKLKSTKEEP

SEQ ID NO: 163 - protein, 726 aa, synthetic construct
SEVEFSHEYWMRHALALAKRARDEREVPVGAVLVLNNRVIGEGWNRAIGLHDPTAHAEIMALRQGGLVMQNYRLTDATLYVTFEPCVMCAGAMIHSRIGRVVFGVRNSKRGAAGSLMNVLNYPGMNHCVEITEGILVDECAALLCDFYRMPRQVLNAQKKAQSSISSGGSSGGSSGSETPGTSESATPEGSGGSSGGSAKNTITKTLKLRIVRPYNSAEVEKIVADEKNSREKIALEKNKDKVKEACSEHLKVAAYCTTQVERNACLFCKARKLDDGFYQKLRGQFPDAVFWQEIGEIFRQLQKQAAEVYNQSLIELYYEIFIKGKGITNASRVEHYLSDVCYTRAAELFKNAAIASGLRSKVRSNFRLKELKNMKSGLPTTKSDNFPIPLVKQKGGQYTGFEISSHNDDFIIKIPFGRWQVKKEIDKYRPWEKFDFEQVRKSPKPISLLLSTQRRKRNKGWSKDEGTEAEIRKVMNGDYQTSYIEVKRGSKIGEKSAWMLNLSIDVPKIDKGVDPSIIGGVDVGVKSPLVCAINNASNRYSISDNDLFRFNKKMFARRRILLKKNRHKRAGHGAKNKLKPISILTGKSERFRKKLIERWACEIADFFVKNKVGTVQMENLESMKRKEDSYFNIRLRGFWPYAEMQNKIEFKLEQYGIKVRKVAPNNTSKTCSKCGHLNNYFNFEYRKKNKFPHFKCEKCNFKENADYNAALNISNPKLKSTKEEP

SEQ ID NO: 164 - protein, 726 aa, synthetic construct
SEVEFSHEYWMRHALTLARRARDEREVPVGAILVLNNRVIGEGWNRAIGLHDPTAHAEIMALRQGGLVMQNYRLIDATLYVTFEPCAMCAGAMIHGRIGRVVFGVRNNKHGAAGSLMNVLNYPGMGHRVEITEGILADECAALLCDFYCMPRQVFNAQKRAQSSINSGGSSGGSSGSETPGTSESATPESSGGGSSGSAKNTITKTLKLRIVRPYNSAEVEKIVADEKNNRERIALEKNKDKVKEACSKHLKVAAYCTTQVERNACLFCKARKLDDKFYQKLRGQFPDAVFWQEIGEIFRQLQKQAAEIYNRSLIELYYEIFIKGKGIANASRVEHYLSDVCYTRAAELFKNAAIASGLRNRIKSNFRLKELKNMKSGLPTTKSDNFPIPLVKQKGGQYTGFEISNHNSDFIIKIPFGRWQAKKEIDKYRPWEKFDFEQVRKSPKPISLLLSTQRRKRNRGWSKDEGTEAEVKKVMNGDYQISYIEVKRGSKIGEKSAWTLNLSIDVPKIDKGVDPSIIGGIDVGVKSPLVCAISNAFSRYSISDNDLFHFNKKMFARRRILLKKSKHKRAGHGVKNKLKPITILTEKSRRFRKKLIERWACEIADFFIKNKVGTVQMENLEGMKRKEDSYFNIRLRGFWPYAEMQNKIEFKLKQYGIEIRKVAPNNTSKTCSKCGHLNNYFNFEYRKKNKFPHFKCERCNFKENADYNAALNISNPKLKSTKEEP

SEQ ID NO: 165 - protein, 726 aa, synthetic construct
SEVEFSHEYWMRHALTLAKRARDEREVPVGAVLVLNNRVIGEGWNRAIGMHDPTAHAEIMALRQGGLVMQNYRLVDATLYVTFEPCVLCAGAMVHSRIGRVVFGVRNSKRGAAGSLMNVLNYPGMNHRVEVTEGILADECAALLCDFYRMPRQVFNARKKAQSSINSGGSSGGSSGSETPGTSESPTPESSGGSPGGSAKNTITKTLKLRIVRPYNSAEVEKIVADEKNNREKIALEKNKDKVKEACSKHLRVAAYCTTQVERNACLFCKARKLDDKFYQKLRGQFPDAVFWQELGEIFRQLQKQAAEIYNQSLIELYYEIFIKGKGIANASSVEHYLSDVCYTRAAELFKNAAIASGLRNKIKSNFRLKELRNMKSGLPTTKSDNFPIPLVRQKGGQYTGFEISNHDGDFIIKIPFGRWQVKEEINKHRPWEKFDFEQVRKSPKPISLLLSTQRRKRNKGWSKDEGTEAEMKKVMNGDYQTSYIEVKRGSKTGEKSAWMLNLSIDVPKIDKGVDPSIIGGIDVGVKSPLVCAINNAFSRYSISDNDLFRFNKKMFARRRILLKKNRHRRAGHGAKNKLKPITILTERSKRFRKKLIERWACEIADFFIKNKVGTVQMENLESMKRKEDSYFNIRLRGFWPYAEMQNRIEFKLKQYGIEIRRVAPNNTSKTCSKCGHLNHYFNFEYRKKNKFPHFKCEKCNFKENADYNAALNISNPKLKSTKEEP

SEQ ID NO: 166 - protein, 726 aa, synthetic construct
SEVEFSHEYWMRHALTLAKRARDEREVPVGAILVLNNRVIGEGWNRAIGLHDPTAHAEIMALRQGGLVTQNYRLIDATLYVTFEPCVMCAGAMIHSRIGRVVFGVRNNKHGAAGSLMNVLNYPGMNHRVEITEGILADECAALLCDFYRMPRQVFNARKKARSSINPGGSSGGSGGSETPGTSESATPENSGGSSGSSAKNTITKTLKLRIVRPYNSAEVEKIVADEKNNREKIALEKNKDKVREACSEHLKVAAYCTTQVEKNACLFCKARKLDDRFYQKLRSQFPDAVFWQEIGEIFRQLQKQAAEIYNQSLIELYYEIFIKGRGFANASSVEHYLSDVCYTRAAELFKNAAIASGLRGKVKSNFRLKELKNMKGGLPTTKSDNFPIPLVKQKGGQYTGFEISSHNDDFIIKIPFGRWQAKKEIDKYRPWEKFDFEQVRKSPKPISLLLSTQRRKRNRGWSKDEGTEAEIRKVMNGDYQTSYIEVKRGSKIGEKSAWMLNLSIDVPKIDKGVDPSIIGGIDVGVKSPLVCAINNAFSRYSISDNDLFRFNKKMFARRRILLGKNRHKRAGHGVKNKLKPITILTEKSGRFRKKLIERWACEIADFFVKNKVGTVQMENLESMKRKEDSYFNIRLRGFWPYAEMQNKIEFKLKQYGIKVRKVAPNNTSKTCSKCGHLNNYFSFEYRKKNKFPHFKCEKCNFKENADYNAALNISNPKLKSTKEEP

SEQ ID NO: 167 - protein, 726 aa, synthetic construct
SEVEFSHEYWMRHALTLAKRARDEREVPVGAVLVLNNRVIGEGWNRAIGLHDPTAHAEIMALRQGGLVMRNYRLTDATLYVTFEPCVMCAGAMIHSRIGRVVFGVRNSKRGAAGSLMNVLNYPGMNHCVEITEGILVDECAALLCDFYRMPRQVLNAQKKAQSSISPGGSSGGSSGSETPGASESVTPKSSGGSSGGSAKNTITKTLKLRIVRPYNSAEVEKIVADEKNNRERIALEKNKDKVREACSKHLKVASYCTTQVERNACLFCKARKLDDKFYQKLRGQFPDAVFWQELGEIFRQLQKQAAEIYNQSLIELYYEIFIKGKGFANASSVEHYLSDVCYTRAAELFKNAAIASGLRGKVKSNFRLKELKNMKSGLPTTKSDNFPIPLVKQKGGQYTGFEISSHNDDFIIKIPFGRWQAKKEIDKYRPWEKFDFEQVRKSPKPISLLLSTQRRKRNKGWSKDEGTEAEIRKVMNGDYQTSYIEVKRGSKIGEKSAWMLNLSIDVPKIDKGVDPSIIGGIDVGVKSPLVCAINNAFSRYSISDNDLFHFNKKVFARRRILLKKNRHKRAGHGVKNKLKSISILTEKSKRFRKKLIERWACEIADFFIKNKVGTVQMENLESMKRKEDSYFNIRLRGFWPYAEMQNKIEFKLKQYGIEIRKVAPNNTSKTCSKCGHLNNYFNFEYRKKNKFPHFKCEKCNFKENADYNAALNISNPKLKSTKEEP

SEQ ID NO: 168 - protein, 726 aa, synthetic construct
SEVEFSHEYWMRHALTLARRARDEREVPVGAVLVLNNRVIGEGWNRAIGLHDPTAHAEIMALRQGGLVMQNYRLTDATLYVTFEPCVMCAGAMIHSRIGRVVFGVRNSKRGAAGSLMNVLSYPGMNHCVEITEGILVDECAALLCDFYRMPRQVLNAQKKARPNINSGGSSGGRSGSETPGTSESATPESSGGSSGGSAKNTITKTLKLRIVRPYNSAEVEKIVADEKNNREKIALEKNKDKVKEACSEHLKVAAYCTTQVERSACLFCKARKLDDKFYQKLRGQFPDAVFWQEIGEIFRQLQKQAAEIYNQSLIELYYEIFIKGKGFANASSVEHYLSDVCYTRAAELFKNAAIASGLRGKVKSNFRLKELKNMKSGLPTTKSDNFPIPLVKQKGGQYTGFEISSHNDDFIIKIPFGRWQVKKEIDKYRPWEKFDFEQVRKSPKPISLLLSTRRRKRNKGWSRDEGTEAEIRKVMNGDYQTSYIEVKRGSKTGEKSAWMLNLSIDVPKIDKGVDPSIIGGIDVGVKSPLVCAINNAFGRYSISDNDLFRFNKKMFARRRILLKKNRHKRAGHGAKNKLKPISILTEKSKRFRKKLIERWACEIADFFIKNKVGTVQIENLESMKRKEDSYFNIRLRGFWPYAEMQNKIEFKLKQYGIKIRKVAPNNTSKTCSKCGHLNNYFNFEYRKKNKFPHFKCEKCYFKEDADYNAALNISNPKLKSTKEEP

SEQ ID NO: 169 - protein, 726 aa, synthetic construct
SEVEFSHEYWMRHALTLAKRARDEREVPVGAVLVLNNRVIGEGWNRAIGLHDPTAHAEIMALRQGGLVLQNYRLVDATLYVTFEPCVLCAGAMVHSRIGRVVFGARNSKRGAAGSLMNILNYPGMNHRVEITEGILADECAALLCDFYRMPRQVFNAQKKAQSSINSGGSSGGSSGGETPSTSESATPESSGGSSGGSAKNTITKTLQLRIVRPYNSAEVEKIVTDEKNNREKIALEKNKDKVKEACSKHLKVAAYCTTQVERNACLFCKARKLDDKFYQKLRGQFPDAVFWQELGGIFRQLQKQAAEIYNQSLIELYYEIFIKGKGITNASRVEHYLSDVCYTRAAELFKNAAIASGLRSKVRSNFRLKELKNMKSGLPTTKSDNFPIPLVKQKGGQYTGFEISSHNSDFIIKIPFGRWQEKEEIDKYRPWEKFDFEQVRKSPKPISLLLSTQRRKKNKGWSKDEGTEAEIRRVMNGDYQTSYIEVKRGSKIGEKSAWMLNLSIDVPKIDKGVDPSIIGGIDVGVKSPLVCAINNAFSRYSISDNDLFHFNKKVFARRRILLKKNRHRRAGHGAKNKLKPITILTEKSKRFRKKLIERWACEIADFFIKNKVGTVQMENLESMKRKEDSYFNIRLRGFWPYAEMQNKIEFKLKQYGIEIRKVAPNNTSRTCSKCGHLNNYFSFEYRKKNKFPHFKCEKCNFKEDADYNAALNISDPKLRSTKEEP

SEQ ID NO: 170 - protein, 726 aa, synthetic construct
SEVEFSHEYWMRHALTLAKRARDEREVPVGAILVLNNRVIGEGWNRAIGLHDPTAHAEIMALRQGGLVMQNYRLIDATLYVTFEPCVMCAGAMIHSRIGRVVFGVRNSKHGAAGSLMNVLNYPGMNHRVEITEGILADECAALLCDFYRMPRQVFSARKKAQSSINPGGSSGGSSGSKTPGTSESATPESSGGSPGGSAKNSITKTLKLRIVRPYNSAEVEKIVADEKNNREKIALEKNKGKVKEACSKHLKVATYCTTQVERNACLFCKARKLDDKFYQKLRGQFPDAVFWQEIGEVFRQLQKQAAEIYNQSLIELYYEIFIKGKGFANASSVEHYLSDVCYTRAAELFKNAAIASGLRGKVKSNFRLKELKNMKSGLPTTKSDNFPIPLVKQKGGQYTGFEISSHNDDFIIKIPFGRWQVKKEINKFRPWEKFDFEQVRKSPKPISLLLSTQRRKRNKGWSRDEGTEAEIRKVMNGDYQTSYIEVKRGSKIGEKSAWMLNLSIDVPKIDKGVDPSIIGGIDVGVKSPLVCAINNAFSRYSISDNDLFHFNKKMFARRRILLRKNRHKRAGHGAKNKLKPITIMTEKSKRFRKKLIERWACEIADFFIKNKVGTVQMENLESMKRKEDSYFNIRLRGFWPYAEMQSKIEFKLRQYGIVVRKVAPNNTSKTCSKCGHLNNYFNFEYRKKNKFPHFKCEKCNFKEDADYNAALNISNPKLKSTKGEP

SEQ ID NO: 171 - protein, 726 aa, synthetic construct
SEVEFSHEYWMRHALTLAKRARDEREVPVGAVLVLNNRVIGEGWNRAIGLHDPTAHAEIMALRQGGLVMQSYRLTDATLYVTFEPCVMCAGAMIHGRIGRVVFGARNSKRGAAGSLMNVLNYPGMNHCVEITEGILVDECAALLCDFYHMPRQVLNAQKKAQSSISSGGSSGSSSGSETPGASESVTPKGSGGSSAGSTKNTITKTLKLRIVRPYNSAEVEKIVADEKNNREKIALEKNKDKVKEACSKHLKVASYCTTQVERNACPFCKARKLDDKFYQKLRGQFPDAVFWQELGEIFRQLQKQAAEIYNQSLIELYYEIFIKGKGFANASSVEHYLSDVCYTRAAELFKNAAIASGLRGKVKSNFRLKELKNMKSGLPTTKSDNFPIPLVKQKGGQYTGFEISSHNDDFIIKIPFGRWQVKKEIDKYRPWEKFDFEQVRKSPKPISLLLSTQRRKRNKGWSKDEGTEAEIKKVMNGDYQISYIEVKRGNKIGEKSAWMLSLSVDVPKIDKGVDPSIIGGIDVGVKSPLVCAINNALSRYSISDNDLFHFNKKMFARRRILLRKNRYKRVGHGTKNKLKPITILTEKSGRFRKKLIERWACEIANFFIKNKVGTVQMENLESMKRKGDSYFNIRLRGFWPYAEMQNKIEFKLKQYGIKIRKVAPNNTSKTCSKCGHLNNYFSFEYRKKNKFPHFKCEKCNFKEDADYNAALNISNPRLKSTKEEP

SEQ ID NO: 172 - protein, 726 aa, synthetic construct
SEVEFSHEYWMRHALTLAKRARDEREVPVGAILVLNNRVIGEGWNRAIGLNDPTAHAEIMALRQGGLVMQNYRLIDATLYVTFEPCVMCAGAMIHSRIGRVVFGVRNNKHGAAGSLVNVLNYPGMNHRVEITEGILADECAALLCDFYRMPRQVFNARKKAQSSINSGGSSGGSSGSETPGTSESATPKSSGGSSGGSAKNTITKTLKLRIVRPYNSAEVEKIVADEKNNREKIALEKNKDKVQEACSKHLKVASYCTTQVERNACPFCKARKLDDKFYQKLRGQFPDAVFWQELGEILRQLQKQAAEIYNQSLIELYYEIFIKGRGFANASSVEHYLSDVCYTRAAELFKNAAIASGLRGKVKSNFRLKELKNMKSGLPTTKSDNFPIPLVKQKGGQYTGFEVSSHNDDFIIKIPFGRWQVKKEIDKYRPWEKFDFEQVRKSPKPISLLLSTQRRKRNKGWSKDEGTEAEIRKVMNGDYQTSYIEVKRGSKTGEKSAWMLNLSIDVPKIDKGVDPSIIGGIDVGVKSPLVCAINNAFSRYSISDNDLFRFNKKMFARRRILLRKNRHKRAGHGAKNKLKPISILTGKSERFRKKLIERWACEIADFFIKNKVGTVQMENLESMKRKEDSYFNIRLRGFWPYAEMQSKIEFKLKQYGIVVRKVAPNNTSKTCSKCGHLNNYFNFEYRKKNKFPHFKCEKCSFKENADYNAALNISNPKLKSTKREP

SEQ ID NO: 173 - protein, 726 aa, synthetic construct
SEVEFSHEYWMRHALTLAKRARDEREVPVGAVLVLNNRVIGEGWNRAIGLHDPTAHAEIMALRQGGLAMQNYRLVDATLYVTFEPCVLCAGAMVHSRIGRVVFGVRNSKRGAAGSLMNVLNHPGMNHRVEITGGILADECAALLCDFYRMPRQVFNAQKKARSNINSGGSSGGSSGSETLGTSESATPESSGGSSGGSAKNTITKTLKLRIVRPYNSAEVEKIVADEKNRREKIALEKNKDKVKEACREHLKVAAYCTTQVERNACLFCKARKLDDKFYQKLRGQFPDAVFWQEISEIFRQLQKQAAEIYNQSLIELYYEIFIKGKGFANASSVEHYLSDVCYTRAAELFRNAAIASGLRGKVKSNFRLKELKNMKSGLPTTKSDNFPIPLVKQKGGQYTGFEISSHNDDFIIKIPFGRWQVKKEIDKYRPWEKFDFEQVRKSPKPISLLLSTQRRKRNKGWSKDEGTEAEIRKVMNGDYQTSYIEVKRGSKIGEKSAWMLSLSIDVPKIDKGVDPSIIGGIDVGVKSPLVCAINNAFGRHSISDNDLFHFNKKMFARRRILLKKNRHRRAGHGAKNKLKPITILTEKSKRFRKKLIERWACEVADFFIKNKVGTVQMENLESMRRREDGYFNIRLRGFWPYAEMQNKIELKLKQYGIKIRKVAPNNTSKTCSKCGHLNDYFNFEYRKKNKFPHFKCEKCNFKEDADYNAALNISNPKLKSTKEEP

SEQ ID NO: 174 - protein, 726 aa, synthetic construct
SEVEFSHEYWMRHALTLARRARDGREVPVGAVLVLNNRVIGEGWNRAIGLHDPTAHAEIMALRQGGLVMQNYRLIDATLYVTFEPCVMCAGAMVHSRIGRVVFGVRNSKRGAAGSLMNVLDYPGMDHRVEITEGILADECAALLCDFYRMPRQVFNAQKKAQSGINSGGSSGGSSGSETPGTSENATPESSGGSSGGSAKNTITKTLQLRIVRPYNSAEVEKIVTDEKNNREKIALEKNKDKVKEACSKHLKVAAYCTTQVERNACLFCKARKLDDKFYQKLRGQFPDAVFWQEIGEIFRQLQRQAAEIYNQSLIELYYEIFIKGKGFANASSVEHYLSDVCYTRAAELFKNAAIASGLRGKIKSNFRLKELKNMKSGLPTTKSDNFPIPLVKQKGGQYTGFEISNHNGDFIIKIPFGRWQVKKEINKYRPWEKFDFEQVRKSPKPISLLLSTQRRKRNKGWSKDEGTEAEIKKVMNGDYQISYIEVKRGSKIGEKSAWTLNLSVDVPKIDKGVDPSIIGGIDVGVKSPLVCAINNALSRYSISDNDLFHFNKKVFARRRILLKKNRHRRAGHGAKNKLKPITILTEKSKRFRKKLIERWACEIADFFIKNKVGIVQMENLESMKRREDSYFNIRLRGFWPYAEMQNKIEFKLKQYGIEIRKVAPNNTSKTCSRCGHLNNYFNFEHRKKNKFPRFKCEKCNFKENADYNAALNISNPKLKSTKEKP

SEQ ID NO: 175 - protein, 726 aa, synthetic construct
SEVEFSHEYWMRRALTLAKRARDEREVPVGAVLVLNNRVIGVGWNRAVGLHDPTAHAEIMALRQGGLVMQNYRLIEATLYVTFEPCIMCAGAMIHSRIGRVVFGVRNSKRGAAGSLMNVLNYPGMNHRVEVTEGILADECAALLCDYYRMPRQVFNARKKAQSSINSGGSSDGGSGNETPGTSESATPESSGGNSGGSAKNTITKTLKLRIVRPYNSAEVEKIVADEKNNREKVALEKNKDKVKEACSKHLKVAAYCTTQVERNACLFCKARKLDDKFYQKLRGQFPDAVFWQEIGEIFRQLQKQAAEIYNQSLIELYYEIFIKGKGFANASSVEHYLSDVCYTRAAELFKNAAIASGLRGKVKSNFRLKELKNMKSGLPTTKSDNFPIPLVKQKGGQYTGFEISSHNDDFIIKVPFGRWQVKKEIDKYRPWEKFDFEQVRKSPKPISLLLSTQRRKRNKGWSKDVGTEAEIRKVMNGDYQTSYIEVKRGSKIGEKSAWMLNLSIDVPKIDKGVDPSIIGGIDVGVKSPLVCAINNAFSRYSISDNDLFRFNKKMFARRRILLRKNRHKRAGHGAKNKLKPITMMTEKSKRFRKKLIERWACEIADFFIKNKVGTVQMENLESMKRKEDSYFNIRLRGFWPYAEMQNKIEFKLKQYGIVVRKVAPNNTSKTCSKCGHLNNYFNFEYRKKNKFPHFKCEKCNFKEDADYNAALNISNPKLKSTKGEP

SEQ ID NO: 176 - protein, 726 aa, synthetic construct
SEVEFSHEYWMRHALTLAKRARDEREVPVGAVLVLNNRVIGEGWNRAIGLHDPTAHAEVMALRQGGLVMQNYRLTDATLYVTFEPCVMCAGAMIHSRIGRVVFGVRNSKRGAAGSLMNVLNYPGMNHRVEITEGILVDECAALLCDFYRMPRQVLNAQKKAQSGISSGGSSGGSSGSETPGASGSVTPKSSGGSSAGSTKDTITKTLKLRIVRPYNSAEVEKIVADEKNSREKIALEKNKDKVKEACSEHLKVAAYCTTQVERNACLFCKARRLDDKFYQKLRDQFPDAVFWQEIGEIFRQLQKQAAEIYNQSLVELYYEILIKGKGIANASSVEHYLSDVCYTRAAKLFKNAAIASGLRNKIKSNFRLKELRNMKSGLPTTKSDNFPIPLVKQKGGQYTGFEISSHNDDFIIKIPFGRWQVKKEIDKYRPWEKFDFEQVRKSPKPISLLLSTQRRKRNKGWSKDEGTEAEIRKVMSGGYQTSYIEVKRGSKTGERSAWVLNLSIDVPKIDRGVDPSIIGGIDVGVKSPLVCAINNALSRYSISDNDLFHFNKKMFARRRILLKKNGHKRAGHGAKNKLKPITIMTEKSKRFRKKLIERWACEIADFFIKNKVGTVQMENLESMKRKEDSYFNIRLRGFWPYAEMQNKIEFKLKQYGIKVRKVAPNNTSKTCSKCGHLNNYFSFEYRKKNKFPHFKCEKCNFKENADYNAALNISNPKLMGTKEEP

SEQ ID NO: 177 - protein, 726 aa, synthetic construct
SEVEFSHEYWMRHALALAKRARDEREVPVGAVLVLNNRVIGEGWNRAIGLHDPTAHAEIMALRQGGLVMQNYRLIDATLYVTFEPCVMCAGAMVHSRIGRVVFGVRNSKRGAAGSLMNVLDYPGMGHRVEITEGILADECAALLCDFYCMPRQVFNAQKRAQSSINSGGSSGGSSGSDTPGTSESATPESSGGGSSGSAKNTITKTLQLRIVRPYNSAEVEKIVADEKNNREKIALEKNKDKVREACSKHLKVASYCTTQVERNACPFCKARKLDDKFYQRLRGQFPDAVFWQELGEILRQLQKQAAEIYNQSLIELYYEIFIKGRGFANASSVEHYLSDVCYTRAAELFKNAAIASGLRGKVKGNFRLKELKNMKSGLPTTKSDNFPIPLVKQKGGQYTGFEISSHNDDFIIKIPFGRWQVKKEIDKYRPWEKFDFEQVRKSPKPISLLLSTQRRKRNKGWSKDEGTEAEIRKVMNGDYQTSYIEVKRGSKTGEKSAWMLNLSIDVPKIDKGVDPSVVGGIDVGVKSPLVCAINNAFSRYSISDNDLFHFNKKMFARRRILLKKNRHKRAGHGAKNKLKPISILTEKSKRFRKKLIERWACEIADFFIKNKVGTVQMENLESMKRKEDSYFNIRLRGFWPYAEMQNKIEFKLKQYGIEIRKVAPNNTSKTCSKCGHLNNYFNFEYRRKNKFPHFKCEKCNFKEDADYNAALNISNPKLKSTKEEP

SEQ ID NO: 178 - protein, 726 aa, synthetic construct
SEVEFSHEYWMRHALTLAKRARDEREVPVGAVLVLNNRVIGEGWNRAIGLHDPTAHAEIMALRQGGLVMQNYRLVDATLYVTFEPCVLCAGAMVHSRIGRVVFGVRNSKRGAAGSLMNVLNYPGMNHRVEITEGILADECAALLCDFYRMPRQVFNARKKAQSSISPGGSSGGSSGSETPGASESVTPKSSGGSSGGPAKNTITKTLKLRIVRPYNSAEVEKIVADEKNNREKIALEKNKGKVKEACSKHLEVAAYCTTQVERNACLFCKARKLDDKFYQKLRGQFPDAVFWQELGEIFRQLQKQAAEIYNQSLIELYYEIFIKGKGFANASSVEHYLSDVCYTRAAELFKNAAIASGLRGKVKSNFRLKELKSMKSGLPTTKSDNFPIPLVKQKGGQYTGFEISSHNDDFIIKIPFGRWQVKKEIDKYRPWEKFDFEQVRKSPKPISLLLSTQRRKRNKGWSKDEGTEAEIRKVMNGDYQTSYIEVKRGSKTGEKSAWMLNLSIDVPKIDKGVDPSIIGGIDVGVKSPLVCAISNAFSRYSISDNDLFRFNKKMFARRRILLKKNRHKRVGHGARNKLKPISILTGKSERFRKKLIERWACEIADFFIKNKVGTVQMENLESMKRKEDSYFNIRLRGLWPYAEMQNKIEFKLKQYGIKIRKVAPNNTSKTCSKCGHLNNYFSFEYRKKNKFPHFKCEKCNFKEDADYNAALNISNPKLKSTKEEP

SEQ ID NO: 179 - protein, 726 aa, synthetic construct
SEVEFSHEYWMRHALTLAKRARDEREVPVGAILVLNNRVIGVGWNRAIGLHDPTAHAEIMALRQGGLVMQNYRLIDATLYVTFEPCVMCAGAMIHSRIGRVVFGVRNSKHGAAGSLVNVLNYPGMNHRIEITEGILADECAALLCDFYRMPRQVFNARKKAQSSINSGGSSGGSSGSETPGTSESATPKNSGGSSGGSAKNTITKALKLKIVRPYNSAEVEKIVADEKNNRERIALEKNKDKVKEACCKHLKVAAYCTTQVERNACLFCKARKLDDKFYQKLRGQFPDAVFWQELGEILRQLQKQAAEIYNQSLIELYYEIFVKGKGFANASSVEHYLSDVCYTRAAELFKNAAIASGLRGKVKSNFRLKELRSMRSGLPTTKSDNFPIPLVKQKGGQYTGFEISSHNDDFIIKIPFGRWQVKKEIDKYRPWEKFDFEQVRKSPKPISLLLSTQRRKRNKGWSKDEGTEAEIRKVMNGDYQTSYIEVKRGSKVGEKSAWMLSLSIDVPKIDKGVNPSIIGGIDVGVKSPLVCAINNALSRYSVSDNDLFRFNKKMFARRRILLKKNRHKRAGHGAKNKLKPITILTKKSERFRKKLIERWACEIADFFIKNKVGTVQMENLESMKRKEDSYFNIRLRGFWPYAEMQNKIEFKLKQYGIEIRKVAPNNTSKTCSKCGHLNNYFNFEYRKRNKFPHFKCEKCNYKEDADYNAALNISNPKLKSTKEEP

SEQ ID NO: 180 - protein, 726 aa, synthetic construct
SEVEFSHEYWMRHALSLAKRARDEREVPVGAVLVLNNRIIGEGWNRAIGQHDPTAHAEIMALRQGGLVMQNNRLTDATLYVTFEPCVMCAGAMIHSRIGRVVFGVRNSKRGAAGSLMNVLNYPGVNHCVEITEGILVDECAALLCDFYRMPRQVLNAQKKAQSSISSGGSSGGCSGSEMPGASESVTPKSSGGSSGGSAKNTITKTLKLRIVRPYNSAEVEKIVADEKNNREKIALEKNKDKVKEACSKHLKVAAYCTTQVERNACLFCKARRLDDKFYQKLRGQFPDAVFWQEIGEIFRQLQKQAAEIYNQSLIELYYEIFIKGKGIANASSVEHYLSDVCYTRAAELFKNAAIASGLRNKVKSNFRLKELRSMKSGLPTTKSDNFPIPLVRQKGGQYTGFEISNHNSDFIIKIPFGRWQAKKEIDKYRPWEKFDFEQVRKSPKPISLLLSTQRRKRNWGWSKDESTEAEIKKVMNGDYQTSYIEVKRGSKVGEKSAWMLNLSIDVPKIDKGVDPSIIGGIDVGVKSPLVCAINNAFSRYSISDNDLYRFNKKMFARRRILLKKNRHRRAGHGAKNKLKPITILTEKSKRFRKKLIERWACEIADFFVKNKVGTVQMENLESMKRKEDSYFNIRLRGFWPYAEMQNKIEFKLKQYGIEIRKVAPNNTSKTCSKCGHLNNYFNFEYRKRNKFPHFKCEKCNFKENADYNAALNICNPKLKSTKEEP

SEQ ID NO: 181 - protein, 726 aa, synthetic construct
SEVEFSHEYWMRHALTLAKRARDEREVPVGAVLVLNNRVIGEGWNRAIGLHDPTAHAEIMALRQGGLVMQNYRLTGATLYVTFEPCVMCAGAMIHSRIGRVVFGVRNSKRGAAGSLMNVLSYPDMNHCVEITEGILVDECAALLCDFYRMPRQVLNAQKRAQSSISSGGSSGGNSGSETPGASESATPKSSGGSSAGSTKNTITKTLKLRIVRPYNSAEVEKIVADEKDNRERIALEKNKDKVKEACSKHLKVAAYCTTQVERNACLFCKARKLDDKFYQKLRGQFPDAVFWQEIGEIFRQLQRQAAEIYNQSLIELYYEIFIKGKGFANASSVEHYLSDVCYTRAAELFKNAAIASGLRGKVKSNFRLKELKNMKSGLPTTKSDNFPIPLVKQKGGQYTGFEISSHNGDFIIKIPFGRWQAKKEIDKYRPWEKFDFEQVRKSPKPISLLLSTQRRKRNKGWSKDEGTEAEIKKVMNGDYQTSYIEVKRGSKVGEKSAWMLNLSIDVPKIDKGVDPSIIGGIDVGVKSPLVCAINNAFSRYSISDNDLYRFNKKMFARRRILLKKSKHRRAGHGAKNKLKPITILTEKSGRFRKKLIERWACEIADFFIKNKVGTVQMENLEGMKRKEDSYFNIRLRGFWPYAEMQNKIEFKLKQYGIEIRKVAPNNTSKTCSKCGHLNNYFNFEYRKKNKFPHFKCEKCNFKENADYNAALNISNPKLKSTKEEP

SEQ ID NO: 182 - protein, 726 aa, synthetic construct
SEVEFSHEYWMRHALTLAKRARDEREVPVGAVLVLNNRVIGEGWNRTTGLHDPTAHAEIMALRQGGLVMQNHRLVDATLYVTFEPCVMCAGAMIHSRIGRVVFGVRNNKHGAAGSLVNVLNYPGMNHRVEITEGILADECAALLCDFYRMPRQVFNARKKAQSSINPGGSSGSSSGSETPGASGSVTPKSSGGSSAGSTKDTITKTLKLRIVRPYNSAEVEKIVADEKNNREKIALEKNKGKVKEACSKHLEVAAYCTTQVERNACLFCKARKLDDGFYQKLRGQFPDAVFWQEIGEIFRQLQKQAAETYNQSLIELYYEIFIKGKGIANASRVEHYLSDVCYTRAAELFKNAAIASGLRNKIKSNFRLRELRNMKSGLPTTKSDNFPIPLVKQKGGQYTGFEISNHDSDFIIKIPFGRWQAKKEIDKYRPWEKFDFEQVRKSPKPISLLLSTQRRKRNRGWSKDEGTEAEIKKVMNGDYQTSYIEVKRGSKIGEKSAWMLNLSIDVPKIDKGVDPSIIGGIDVGVKSPLVCAINNAFSRYSISDNDLFHFNKKMFARRRILLKKSRHKRAGHGAKNKLKPITILTEKSKRFRKKLIERWACEIADFFIKNKVGTVQMENLESMKRKEDSYFNIRLRGFWPYAEMQNKIEFKLKQYGIVVRKVAPNNTSKTCSKCGHLNNYFNFEYRKKNKFPHFKCEKCNFKEDADYNAALNISNPKLKSTKGEP

SEQ ID NO: 183 - protein, 726 aa, synthetic construct
SEVEFSHEYWMRHALTLAKRARDEREVPVGAILVLNNRVIGVGWNRAIGLHDPTAHAEIMALRQGGLVMQNYRLIDATLYVTFEPCVMCAGAMIHSRIGRVVFGVRNNKHGAAGSLVNVLNYPGMNHRVEITEGILADECAALLCDFYRMPRQVFNARKKAQSNINSGGSSGGSSGSEAPGTSESPTPESSGGSSGGSVKNTITKTLKLRIVRPYNSAEVEKIVADEKNNREKIALEKNKDKVKEACSKHLKVAAYCTTQVERNACLFCKARKLDDKFYQKLRGQFPDAVFWQEIGEIFRQLQRQAAEIYNQSLIELYYEIFIKGKGFANASSVEHYLSDVCYTRAAELFKNAAIASGLRGKVKSNFRLKELKNMKSGLPTTKSDNFPIPLVKQKGGQYTGFEISSHNDDFIIKIPFGRWQVKKEIDKYRPWEKFDFEQVRKSPKPISLLLSTQRRRRSKGWSKDEGTEAEIRKVMNGDYQTSYIEVKRGSKIGEKSAWMLSLSIDVPKIDKGVDPSIIGGIDVGVKSPLVCAINNALSRYSISDNDLFHFNKKMFARRRILLRKNRHKRAGHGAKNKLKPITMMTEKSKRFRKKLIERWACEIADFFIKNKVGTVQMENLESMKRKEDSYFNIRLRGFWPYAEMQNKIEFKLKQYGIVVRKVAPNNTSKTCSKCGHLNNYFNFEYRKKNKFPHFKCEKCNFKENADYNAALNISNPRLKSTKEEP

SEQ ID NO: 184 - protein, 726 aa, synthetic construct
SEVEFSHEYWMRRALTLAKRARDEREVPVGAVLVLNNRVIGVGWNRAVGLHDPTAHAEIMALRQGGLVMQNYRLTDATLYVTFEPCVMCAGAMIHSRIGRVVFGVRNSKRGAAGSLMNVLNYPGMNHRVEITEGILVDECAALLCDFYRMPRQVLNAQKKAQSSISSGGSSGGSSGNETPGASESATPKSSSGSSAGSTKNTITKTLKLRIVRPYNSAEVEKIVADEKNNREKIALEKNKDKVKEACSKHLKVASYCTTQVERNACPFCKARKLDDKFYQKLRGQFPDAVFWQELGEILRQLQKQAAEIYNQSLIELYYEIFIKGRGFANASSVEHYLSDVCYTRAAELFKNAAIASGLRGKVKSNFRLKELKNMKSGLPTTKSDNFPIPLVKQKGGQYTGFEISSHNDDFIIKIPFGRWQVKKEIDKYRPWEKFDFEQVRKSPKPISLLLSTQRRKRNRGWSKDEGTEAEIRKVMNGDYQTSYIEVKRGRKIGEKSVWMLNLSIDVPKIDKGVDPSTIGGIDVGVKSPLVCAINNAFSRYSISDNDLFRFNKKMFARRRILLKKNRHKRAGHGAKNKLKPITILTEKSGRFRKKLIERWACEIADFFIKNKVGTVQMENLESMKRKEDSYFNIRLRGFWPYAEMQNKIELKLKQYGIKIRKVAPNNTSKTCSKCGHLNDYFNFEYRKKNKFPHFKCEKCNFKEDADYNAALNISNPKLKSTREEP

SEQ ID NO: 185 - protein, 726 aa, synthetic construct
SEVEFSHEYWMRHALTLAKRARDEREVPVGAILVLNNRVIGVGWNRAIGLHDPTAHAEIMALRQGGLVMQNYRLIDATLYVTFEPCVMCAGAMIHSRIGRVVFGVRNSKHGAAGSLVNVLNYPGMNHRVEITEGILADECAALLCDFYRMPRQVFNARKKAQSSINSGCSSGGSSGSETPGTSESATPESSGGGSSGSAKNTITKTLQLRIVRPYNSAEVEKIVADEKNNREKIALEKNKGKVKEACSKHLKVAAYCTTQVERSACQFCKARKLDDKFYQKLRGQFPDAVFWQEIGEIFRQLQKQAAEIYNQSLIELYYEIFIKGKGFANASSAEHYLSDVCYTRAAELFKNAAIASGLRGKVKSNFRLKELKNMKSGLPTTKSDNFPIPLVKQKGGKYTGFEISSHNDDFIIKIPFGRWQVKKEIDKYRPWEKFDFEQVRKSPKPISLLLSTQRRKRNKGWSKDEGTEAEIRKVMNGDYQTSYIEVKRGSKIGEKSAWMLNLSIDVPKIDKGVDPSIIGGIDVGVKSPLVCAINNAFSRYSISDNDLFHFNKKMFARRRILLKKNRHKRAGHGAKNKLKPISILTEKSKRFRKKLIERWACEIADFFIKNKVGTVQMENLESMKRKEDSYFNIRLRGFWPYAEMQNKIEFKLKQYGIEIRKVAPNNTSKTCSKCGHLNNYFNFEYRKMNKFPHFKCEKCNFKENADYNAALNISNPKLKSTKEEP

SEQ ID NO: 186 - protein, 726 aa, synthetic construct
SEVEFSHEYWMRHALALAKRARDEREVPVGAVLVLNNRAIGEGWNRAIGLHDPTAHAEIMALRQGGLVMQNYRLTDATLYVTFEPCVMCAGAMIHSRIGRVVFGVRNSKRGAAGSLMNVLNYPGMNHCVEITEGILADECAALLCDFYRMPRQVLNAQKKAQSSISSGGSSGGSSGSETPGASGSVTPKSSVGSSAGSTKNTITKTLKLRIVRPYNSAEVEKIVADEKNNREKIALEKNRDKVKEACSKHLKVAAYCTTQVERNACLFCKARRLDDKFYQKLRGQFPDAVFWQEIGEIFRQLQKQAAEVYNQSLVELYYEILIKGKGIANASSVEHYLSDVCYTRAAELFKNAAIASGLRNKIKSNFRLKELRNMKSGLPTTKSDNFPIPLVKQKGGQYTGFEISSHNDDFIIKIPFGRWQVKKEFDKYRPWEKFDFEQVRKSPKPISLLLSTQRRKRNKGWSKDEGTEAEIRKVMSGDYQTSYIEVKRGSKTGEKSAWMLNLSIDVPKIDKGVDPRIIGGIDVGVKSPLVCAINNAFSRYSISDNDLFHFNKRMFARRRILLKKNGHKRAGHGTKNKLKPITIMTEKSKRFRKKLIERWACEIADFFIKNKVGTVQMENLESMKRREDSYFNIRLRGFWPYAEMQNKIEFKLKQYGIEIRKVAPNNTSKTCSKCGHLNNYFNFEYRKKNKFPHFKCEKCNFKENADYNAALNISNPKLKSTKEKP

SEQ ID NO: 187 - protein, 726 aa, synthetic construct; identical to SEQ ID NO: 92

SEQ ID NO: 188 - protein, 726 aa, synthetic construct
SEVGFSHEYWMRHALTLAKRARDEREVPVGAVLVLNNRVIGEGWNRAIGLHDPTAHAEIMALRQGGLVMQNYRLVDATLYVTFEPCVMCAGAMIHSRIGRVVFGVRNNKHGAAGSLVNVLNYPGMNHRVEITEGILADECAALLCDFYRMPRQVFNGRKKAQSSINSGGSSGGSSGSETPGTSESATPESSGGSSSGSTKNTITKTLKLRIVRPYNSTEVEKIVADEKNNREKIALEKNKDKVKEACSKHLKVAAYCTTQVERNACLFCKARKLDDKFYQKLRGQFPDAVFWQELGEIFRQLQKQAAEIYNQSLIELYYEIFIKGRGFANAGSVEHYLSDVCYTRAAELFKNAAIASGLRGKVKSNFRLKELKNMKSGLPTTKSDNFPIPLVKQKGGQYTGFEISSHNDDFIIKIPFGRWQVKKEIDKYRPWEKFDFEQVRKSPKPISLLLSTQRRKRNKGWSKDEGTEAEIRKVMNGDYQTSYIEVKRGSKTGEKSAWMLNLSIDVPKIDKGVDPSIIGGIDVGVKSPLVCAINNALSRYSISDNDLFRFNKKMFARRRILLKKNRHKRAGHGAKNKLKPISILTGKGERFRKKLIERWACEIADFFIKNKVGTVQMENLESMKRKEDSYFNIRLRGFWPYAEMQNKIEFKLKQYGIEIRKVAPNNTSKTCSKCGHLNSYFNFEYRKKNKFPHFKCEKCNFKENADYNAALNISNPKLKSTKEEP

SEQ ID NO: 189 - protein, 726 aa, synthetic construct
SEVGFSHEYWMRHALTLAKRARDEREVPVGAVLVLNNRVIGEGWNRAIGLHDPTAHAEIMALRQGGLVMQNYRLTDATLYVTFEPCVMCAGAMVHSRIGRVVFGVRNSKRGAAGSLMNVLDYPGMGHRVEITEGILADECAALLCDFYCMPRQVFNAQRRAQSSINSGGSSGGSSGSETPGTSESVTPKSSGGSSAGSTKNTITKTLKLRIVRPYNSAEVEKVVADEKNSREKIALEKNKDKVKEACSEHLKVAAYCTTQVERNACLFCKARKLDDRFYQKLRGQFPDAVFWQEIGEIFRQLQKQAAEIYNQSLIELYYEIFIKGKGFANASSVEHYLSDVCYTRAAELFKNAAIASGLRGKVKSNFRLKELKNMKSGLPTTKSDNFPIPLVRQKGGQYTGFEVSSHNDDFIIKIPFGRWQVKKEIDKYRPWEKFDFEQVRKSPRPISLLLSTQRRKRNKGWSRDEGTEAEIRKVMNGDYQTSYIEVKRGSKIGEKSAWMLNLSIDVPKIDKGVDPSIIGGIDVGVKSPLVCAIDNAFSRYSISDNDLFRFNKKMFARRRILLGKNRHKRAGHGVKNKLKPITILTEKSGRFRKKLIERWACEIADFFVKNKVGTVQMENLESMKRKEDSYFNIRLRGFWPYAEMQNKIEFKLKQYGIKVRKVAPNNTSKTCSKCGHLNNYFSFEYRKKNKFPHFKCERCNFKENADYNAALNISNPKLKSTKEEP

SEQ ID NO: 190 - protein, 726 aa, synthetic construct
SEVEFSHEYWMRHALTLAKRARDEREVPVGAVLVLNNRVIGEGWNRAIGLHDPTAHAEIMALRQGGLVMQNYRLIDATLYVTFEPCVMCAGAMIHSRIGRVVFGVRNSKHGAAGSLVNVLNYPGMNHRVEITEGILADECAALLCDFYRMPRQVFNARKKAQSSINPSGLSGGSSGSETPGASESVTPKSSGGSSGGSAKNTITKTLKLRIVRPYNSAEVEKIVADEKNNREKIALEKNKDKVKEACSKHLKVAAYCTTQVERNACLFCKARRLDDKFYQKLRGQFPDAVFWQEIGEIFRQLQKQAAEIYNQSLIELYYEIFIKGKGFANASSVEHYLSDVCYTRAAELFKNAAIASGLRGKVKSNFRLKELKNMRSGLPTTKSDNFPIPLVKQKGGQYAGFEISSHNDDFIIKIPFGRWQVKKEIDKYRPWEKFDFEQVRKSPKPISLLLSTQRRKRNKGWSKDEGTEAEIRKVMNGDYQTSYIEVKRGSKIGEKSAWMLSLSIDVPKIDKGVDPRTIGGIDVGVKSPLVCAINNVLSRYSISDNDLFHFNKKMFARRRILLKKNGHKRAGHGAKNKLKPITLMTEKSKRFRKKLIERWACEIADFFIKNKVGTVQMENLESMKRKEDSYFNIRLRGFWPYAEMQNKIEFKLKQYGIVVRKVAPNNTSKTCSQCGHLNNYFSFEYRKKNKFPHFKCEKCNFKEDADYNAALNISNPKLKSTKEEP

SEQ ID NO: 191 - protein, 726 aa, synthetic construct
SEVEFSHEYWMRHALTLAKRARDEREVPVGAVLVLNNRVIGEGWNRAIGLHDPTAHAEVMALRQGGLVMQNYRLTDATLYVTFEPCVMCAGAMIHSRIGRVVFGVRNSKRGAAGSLMNVLNYPGMNHCVEITEGILVDECAALLCDFYRMPRQVLNAQKKAQSSISSGGSSGGSSGSVTPGASGSVTPKSSGGSSAGSTKDTITKALKLRIVRPYNSAEVEKIVADEKNNRERIALEKNKDKVKEACSKHLKVAAYCTTQVERNACLFCKARKLDDKFYQKLRGQFPEAVFWQEIGEIFRQLQKQAAEIYNQSLIELYYEIFIKGKGFANASSVEHYLSDVCYTRAAELFKNAAIASGLRGKVKSNFRLKELKNMKSGLPTTKSDNFPIPLVKQKGGQYTGFEISSHNDDFIIKIPFGRWQVKKEIDKYRPWEKFDFEQVRKSPKPISLLLSTQRRKRNEGWSKDEGTEAEIRKVMNGDYQTSYIEVKRGSKIGEKSTWMLNLSIDVPKIDKGVDPSIIGGIDVGVKSPLVCAIDNAFSRYSISDNDLFHFNKKMFARRRILLKKNRHKRAGHGAKNKLKPISILTEKSKRFRKKLIERWACEIADFFVKNKVGTVQMENLESMKRKEDSYFNIRLRGLWPYAEMQNKIEFKLKQYGIEIRKVAPNNTSKTCSKCGHLNNYFNFEYRKKNKFPHFKCEKCNFKENADYNAALNISNPKLKSTKEEP

SEQ ID NO: 192 - protein, 726 aa, synthetic construct
SEVEFSHEYWMRHALALAKRARDEREVPVGAVLVLNNRAIGEGWNRAIGLHDPTAHAEIMALRQGGLVMQNYRLTDATLYVTFEPCVMCAGAMIHSRIGRVVFGVRNSKRGAAGSLMNVLNYPGMNHCVEITEGILVDECAALLCDFYRMPRQVLNAQKKAQSSISSGGSSGGCSGSEMPGASESVTPKSSGGSSAGSTKNTITKTLKLRIVRPYNSAEVEKIVADEKNSREKIALEKNKDKVKEACSEHLKVAAYCTTQVERNACLFCKARKLDDKFYLKLRGQFPDAVFWQEIGEIFRQLQKQAAEIYNQSLIELYYEIFIKGKGITNASRVEHYLSDVCYTRAAELFKNAAIASGLRSKVRSNFRLKELKSMKSGLPTTKSDNFPIPLVKQKGGQYTGFEIRSHNSDFIIKIPFGRWQVKEEIDKYRPWEKFDFEQVRKSPKPISLLLSTQRRKRNKGWSKDEGTEAEIRKVMNGDYRTSYIEVKRGSKIGEKSAWMLNLSIDVPKIDKGVDPSIIGGIDVGVKSPLVCAINNALSRYSISDNDLFHFNKKVFARRRILLKKNRHRRAGHGAKNKLKPITILTEKSKRFRKKLIERWACEIADFFIKNKVGIVQMENLESMKRREDSYFNIRLRGFWPYAEMQNKIEFKLKQYGIKVRKVAPNNTSKTCSKCGHLNNYFSFEYRKKNKFPHFKCEKCNFKENADYNAALNISNPKLKSTKEEP

SEQ ID NO: 193 - protein, 726 aa, synthetic construct
SEVEFSHEYWMRHALTLAKRARDEREVPVGAILVLNNRVIGEGWNRAIGLNDPTAHAEIMALRQGGLVMQNYRLIDATLYVTFEPCVMCAGAMIHSRIGRVVFGVRNNKHGAAGSLVNVLNYPGMNHRVEITEGILADECAALLCDFYRMPRQVFNAQKKARSNINSGGSSGGSSDSETPGTSESATPESSGGSSGGSAKNTITKTLKLRIVRPYNSAEVEKIVADEKNNREKIALEKNKDKVKEACSKHLKVASYCTTQVERNACLFCKARKLDDKFYQKLRGQFPDAVFWQELGGIFRQLQKQAAEIYNQSLIELYYEIFIKGKGITNASRVEHYLSDVCYTRAAELFKNAAIASGLRSKVRSNFRLKELKNMKSGLPTTKSDNFPIPLVRQKGGQYTGFEISSHNSDFIIKIPFGRWQVKEEIDKYRPWEKFDFEQVRKSPKPISLLLSTQRRKKNKGWSKDEGTEAEIRRVMNGDYRTSYIEVKRGSKIGEKSAWMLNLSIDVPKIDKGVDPSIIGGIDVGVKSPLVCAINNSLSRYSICDNDLFRFNKKMFARRRILLKKNRHKRAGHGAKNKLKPITILTKKSERFRKKLIERWACEVADFFIKNKVGTVQMENLESMKRKEDSYFNIRLRGFWPYAEMQDRIEFKLKQYGIEIRRVAPANTSRTCSKCGHLNNYFNFEYRKENKFPHFKCEKCNFREDADYNAALNISSPKLKSTKEEP

SEQ ID NO: 194 - protein, 726 aa, synthetic construct
SEVEFSHEYWMRHALTLAKRARDEREVPVGAVLVLNNRVIGEGWNRAIGLHDPTAHAEIMALRQGGLVMQNYRLIDATLYVTFEPCVMCAGAMIHSRIGRVVFGVRNNKRGAAGSLMNVLNYPGMNHRVEITEGILADECAALLCDFYCMPRQVLNAQKKARSCINSGGSSGGSSGSETPGTSESATPESSGGSSGGSAKNTITKTLKLRIVRPYNSAEVEKIVADEKDNRERIALEKNKGKVKEACSKHLKVAAYCTTQVERNACLFCKARKLDDKFYQELRGQFPDAVFWQELGEILRQLQKQAAEIYNQSLIELYYEIFIKGRGFANASSVEHYLSDVCYTRAAELFKNAAIASGLRGKVKSNFRLKELKNMKSGLPTTKSDNFPIPLVKQKGGQYTGFEISSHNSDFIIKIPFGRWQMKEEIDKYRPWEKFDFEQVRKSPKPISLLLSTQRRKKNKGWSKDEGTEAEIRRVMNGDYQTSYIEVKRSSKIGEKSAWMLNLSIDVPKIDKGVDPSIVGGIDVGVKSPLVCAINNSFSRYSICDNDLFRFNKKVFARRRILLKKNKHRRAGHGAKNKLKPITILTEKSKRFRKKLIERWACEIADFFIKNKVGTVQMENLESMKRKEDSYFNIRLRGFWPYAEMQNKIEFKLKQYGVKVRKVAPNNTSRTCSRCGHLNNYFSFEYRKKNKFPHFKCEKCNFREDADYNAALNISNPKLKSTKGEP

SEQ ID NO: 195 - protein, 726 aa, synthetic construct
SEVEFSHEYWMRHALTLAKRARDEREVPVGAVLVLNNRVIGEGWNRAIGLHDPTAHAEIMALRQGGLVMQNYRLTDATLYVTFEPCVMCAGAMIHSRIGRVVFGVRNSKRGAAGSLMNVLNYPGMNHRVEITEGILVDECAALLCDFYRMPRQVLNAQKKAQSSISPGGSSGGSSGSETPGASGSVTPKSSGGSSAGSTKDTITKTLKLRIVRPYNSAEVEKIVADEKNSREKIALEKNKDKVKEACSEHLKVAAYCTTQVERNACLFCKARKLDDRFYQKLRGQFPDAVFWQEIGEIFRQLQKQAAEIYNQSLIELYYEIFIKGKGFANAGSVEHYLSDVCYTRAAELFKNAAIASGLRGKVKSNFRLKELKNMKSGLPTTKSDNFPIPLVKQKGGQYTGFEISSHNDDFIIKIPFGRWQVKKEIDKYRPWEKFDFEQVRKSPKPISLLLSTQRRKRNKGWSKDEGTEAEIRKVMNGDYQTSYIEVKRGSKIGEKGAWMLNLSIDVPKIDKGVDPSIIGGIDVGVKSPLVCAINNAFSRYSIGDNDLFHYNKKMFARRRILLKKNRHKRAGHGAKNKLKPISILTEKSKRFRKKLIERWACEIADFFIKNKVGTVQIENLESMKRKEDSYFNIRLRGFWPYAEMQNKIEFKLKQYGIEIRKVAPNNTSKTCSKCGHLNSYFNFEYRKKNKFPHFKCEKCNFKENADYNAALNISNPKLKSTKEEP

SEQ ID NO: 196 - protein, 726 aa, synthetic construct
SEVEFSHEYWMRHALTLAKRARDEREVPVGAILVLNNRVIGEGWNRAIGLHDPTAHAEIMALRQGGLVMQNYRLIDATLYVTFEPCVMCAGAMIHSRIGRVVFGVRNSKHGAAGSLVNVLNYPGMNHRVEITEGILADECAALLCDFYRMPRQVFNARKKAQSSINPSGSSGGSSGSVTPGTSESATPESSGGGFGGSAKNTITKTLKLRIVRPYNSAEVEKIVADEKNYRERIALEKNKDKVKEACSKHLKVATYCTTQVERNACLFCKARRLDDKFYQKLRGQFPDAVFWQEIGEIFRQLQKQAAEIYNQSLVELYYEIFIKGKGIANASSVEHYLSDVCYTRAAELFKNAAIASGLRNKIKSNFRLKELRNMKSGLPTTKSDNFPIPLVRQKGGQYTGFEISNHDGDLIIKIPFGRWQVKKEINKHRPWEKFDFEQVRKSPKPISLLLSTQRRKRNKGWSKDEGTEAEIRKVMNGDYQTSYIEVKRGSKIGEKSAWMLNLSIDVPRIDKGVDPSIIGGIDVGVKSPLVCAINNALSRYSISDNDLFHFNKKMFARRRILLRKNRHKRAGHGAKNKLKPITIMTEKSKRFRKKLIERWACEIADFFIRNKVGTVQMENLESMKRKEDSYFNIRLRGFWPYAEMQNKIEFKLKQYGIVVRKVAPNNTSKTCSKCGHLNNHFNFEYRKKNKFPHFKCEKCNFKEDADYNAALNISNPKLKSTKGEP

SEQ ID NO: 197 - protein, 726 aa, synthetic construct
SEVEFSHEYWMRHALTLAKRARDEREVPVGAVLVLNNRVIGEGWNRAIGLHDPTAHAEIMALRQGGLVMQNYRLTDATLYVTFEPCVMCAGAMIHSRIGRVVFGVRNSKRGAAGSLMNVLNYPGMNHCVEITEGILVDECAALLCDFYRMPRQVLNAQKKAQSSISSGGSSGGSSGSETPGTSESPTPESSGGSPGGSAKNTITKTLKLRIVRPYNSAEVEKIVADEKDNREKIALEKNKDKVKEACSKHLKVAAYCTTQVERNACLFCKARKLDDKFYQKLRGQFPDAVFWQEIGEIFRQLQKQAAEIYNQSLIELYYEIFIKGKGFANASSVEHYLSDVCYTRAAELFKNAAIASGLRGKVKSNFRLKELKNMKSGLPTTKSDNFPVPLVKQKGGQYTGFEISSHNDDFIIKIPFGRWQVKEEIDKYRPWEKFDFEQVRKNPKPISLLLSTQRRKRNKGWSKDEGTEAEIRKVMNGDYQTSYIEVKRGSKIGEKSAWMLNLSIDVPKIDKGVDPSIIGGIDVGVKSPLVCAINNAFSRYSISDNDLFRFNKKVFARRRILLKKNRHKRAGHGTKNKLKPITILTEKSGRFRKKLIERWACEIANFFIKNKVGTVQMENLESMKRKGDSYFNIRLRGFWPYAEMQNKIEFKLKQYGIKIRKVAPNNTSKTCSKCGHLNNYFSFEYRKKNKFPHFKCEKCNFKEDADYNAALNISNPKLKSTKEEP

SEQ ID NO: 198 - protein, 726 aa, synthetic construct
SEVEFSHEYWMRHALTLAKRARDEREVPVGAVLVLNNRVIGEGWNRAIGLHDPTAHAEVMALRQGGLVMQNYRLTDATLYVTFEPCVMCAGAMIHSRIGRVVFGVRNSKRGAAGSLMNVLNYPGMNHRVEITEGILVDECAALLCDFYRMPRQVLNAQKKAQSSISPGGSSGGSSGSETPGASGSVTPKSSGGSSAGSTKDTITKTLKLRIVRPYNSAEVEKIVADEKNSREKIALEKNKDKVKEACSEHLKVAAYCTTQVERNACLFCKARKLDDRFYQKLRGQFPDAVFWQEIGEIFRQLQKQAAEVYNQSLVELYYEILIKGKGIANASSVEHYLSDVCYTRAAELFKNAAIASGLRNKIKSNFRLKELRNMKSGLPTTKSDNFPIPLVRQKGGQYTGFEISNHDGDFIIKIPFGRWQVKKEINKHRPWEKFDFEQVRRSPKPISLLLSTQRRKRNKGWSKDEGTEAEIRKVMNGDYQTSYIEVKRGSKIGEKSAWMLNLSIDVPKIDKGVDPSIIGGIDVGVKSPLVCAINNALSRYSISDNDLFHFNKKMFARRRILLRKNRHKRAGHGAKNKLKPISILTEKSKRFRKKLIERWACEIADFFIKNKVGTVQMENLESMKRKEDSYFNIRLRGFWPYAEMQNKIEFKLKQYGIEIRKVAPNNTSKTCSKCGHLNNYFNFEYRKKNKFPHFKCEKCNFKENADYNAALNISNPKLKSTKEEP

SEQ ID NO: 199 - protein, 726 aa, synthetic construct
SEVEFSHEYWMRHALTLAKRARDEREVPVGAVLVLNNRVIGEGWNRAIGLHDPTAHAEIMALRQGGLVVQNYRLTDATLYVTFEPCVMCAGAMIHSRIGRVVFGVRNSKRGAAGSLMNVLNYPGMNHCVEITEGILVDECAALLCDFYRMPRQVLNAQKKAQSSISSGGSSGGSSGSETPGASGSVTPKSSGGSSAGSTKDTITKTLKLRIVRPYNSAEVEKIVADEKNSREKIALEKNKDKVKEACSEHLKVAAYCTTQVERNACLFCKARRLDDKFYQKLRGQFPDAVFWQEIGEIFRQLQKQAAEIYNQSLVELYYEILIKGKGIANASSVEHYLSDVCYTRAAELFKNAAIASGLRNKIKSNFRLKELRNMKSGLPTTKSDNFPIPLVKQKGGQYTGFEINSHNDDFIIKIPFGRWQVKKEIDKYRPWEKFDFEQVRKSPKPISLLLSTQRRKRNKGWSKDEGTEAEIRKVMNGDYQTSYIEVKRGSKTGEKSAWMLNLSIDVPKIDKGVDPSIIGGIDVGVKSPLVCAINNAFSRYSIGDNDLFHYNKKMFARRRILLKKNRLKRAGHGAKNKLKPISILTEKSKRFRKKLIERWACEIADFFIKNKVGTVQMENLESMKRKEDSYFNIRLRGFWPYAEMQNKIEFKLKQYGIEIRKVAPNNTSKTCSKCGHLNNYFNFEYRKKNKFPHFKCEKCNFKENADYNAALNISNPKLKSTKEEP

SEQ ID NO: 200 - protein, 726 aa, synthetic construct
SEVEFSHEYWMRRALTLAKRARDEREVPVGAILVLNNRVIGEGWNRAIGLHDPTAHAEIMALRQGGLVMQNYRLIDATLYVTFEPCVMCAGAMIHSRIGRVVFGVRNNKHGAAGSLVNVLNYPGMNHRVEITEGILADECAALLCDFYRMPRQVFNARKKAQSSINPGGSSGGSSGSETPGTSESATLESSGGSSGGSAKNTITKTLKLRIVRPYNSAEVEKIVADEKNNREKIALEKNKDKVKEACSKHLKVASYCTTQVERNACLFCKARKLDDKFYQKLRGQFPDAVFWQELGGIFRQLQKQAAEIYNQSLIELYYEIFIKGKGITNASRVEHYLSDVCYTRAAELFKNAAIASGLRSKVRSNFRLKELKNMKSGLPTTKSDNFPIPLVKQKGGQYTGFEISSHNSDFIIKIPFGRWQEKEEIDKYRPWEKFDFEQVRRSPKPISLLLSTQRRKRNKGWSKDEGTEAEIRKVMNGDYQTSYIEVKRGSKTGEKSAWMLNLSIDVPKIDKGVDPSIIGGIDVGVKSPLVCAINNAFSRYSIGDNDLFRYNKKMFARRRILLKKNRHKRAGHGAKNKLKPISILTEKSKRFRKKLIERWACEIADFFIKNKVGTVQMENLESMKRKEDSYFNIRLRGFWPYAEMQNKIEFKLKQYGVEIRRVAPNNTSRTCSKCGHLNNYFNFEYRRKNKFPHFKCEKCNFKEDADYNAALNISNPKLKSTREEP

SEQ ID NO: 201 - protein, 726 aa, synthetic construct
SEVEFSHEYWMRHALALAKRARDEREVPVGAVLVLNNRVIGEGWNRAIGLHDPTAHAEIMALRQGGLVMQNYRLIDATLYVTFEPCVMCAGAMVHSRIGRVVFGVRNSKRGAAGSLMNVLDYPGMGHRVEITEGILADECAALLCDFYCMPRQVFNAQKRAQSSINSGGSSGGSSGSETPGTSESATPESSGGGSSGSAKNTITKTLKLRIVRPYNSAEVEKIVADEKNNREKIALEKNKDKVKEACSEHLKVAAYCTTQVERNACPFCKARKLDDKFYRKLRGQFPDAVFWQEIGEIFRQLQKQAAEIYNQSLIELYYEILIKGKGFANASSVEHYLSDVCYTRAAELFKNAAIASGLRGKVKSNFRLKELKNMKSGLPTTKSDNFPIPLVKQKGGQYTGFEISSHHDDFIIKIPFGRWQVKKEIDKYRPWEKFDFEQVRKSPKPISLLLSTQRRKRNKGWSKDEGTEAEIRKVMNGDYQTSYIEVKRGSKTGEKSAWMLNLSIDVPKIDKGVDPSIIGGIDVGVKSPLVCAINNAFSRYSISDNDLFRFNKKMFARRRILLGKNRHKRAGHGVKNKLKPITILTEKSGRFRKKLIERWACEIADFFVKNKVGTVQMENLESMKRKEDSYFNIRLRGFWPYAEMQNKIEFKLKQYGIEIRKVAPNNTSKTCSKCGHLNSYFNFEYRKKNKFPHFKCEKCNFKENADYNAALNISNPKLKSTKEEP

SEQ ID NO: 202 - protein, 726 aa, synthetic construct
SEVEFSHEYWMRHALTLAKRARDEREVPVGAVLVLNNRVIGEGWNRAIGLHDPTAHAEIMALRQGGLVMQNYRLTDATLYVTFEPCVMCAGAMIHSRIGRVVFGVRNSKRGAAGSLMNVLNYPGMNHCVEITEGILVDECAALLCDFYRMPRQVLNAQKKAQSSISPGGSSGGSSGSETPGASGSVTPKSSGGSSAGSTKDTITKTLKLRIVRPYNSAEVEKIVADEKNSREKIALEKNKDKVKEACSEHLKVAAYCTTQVERNACLFCKARKLDDRFYQKLRGQFPDAVFWQEIGEIFRQLQKQAAEIYNQSLIELYYEIFIKGKGFANASSVEHYLSDVCYTRAAELFKNAAIASGLRGKVKSNFRLKELKNMKSGLPTTKSDNFPIPLVKQKGGQYTGFEISSHNDDFIIKIPFGRWQVKKEIDKYRPWEKFDFEQVRKSPKPISLLLSTQRRKKNKGWSKDEGTEAEIRRVMNGDYQTSYIEVKRGSKIGEKSAWMLNLSIDVPKIDKGVDPSIIGGIDVGVKSPLVCAINNAFSRYSISDNDLFRFNKKMFARRRILLKKNRHQRAGHGAKNKLKPITILTEKSGRFRKKLIERWACEIADFFIKNKVGTVQMENLESMKRKEDSYFNIRLRGFWPYAEMQSKIEFKLKQYGIEIRKVAPNNTSKTCSKCGHLNNYFNFEYRKMNKFPHFKCEKCNFKENADYNAALNISNPKLKSTKEEP

SEQ ID NO: 203 - protein, 726 aa, synthetic construct
SEVEFSHEYWMRHALTLAKRARDEREVPVGAVLVLNNRVIGEGWNRAIGLHDPTAHAEIMALRQGGLVLQNYRLVDATLYVTFEPCVLCAGAMVHSRIGRVVFGARNSKRGAAGSLMNILNYPGMNHRVEITEGILADECAALLCDFYRMPRQVFNAQKKAQSSINSGGSSGGSSGSGTLGTSGSPTRESFGGSSGGSAKNTITKTLKLRIVRPYNSAEVEKIVADEKNNREKIALEKNRGKVKEACSKHLKVAAYCTTQVERNACLFCKARKLDDKFYQKLRGQFPDAVFWQEIGEIFRQLQKQAAEIYNQSLIELYYEIFIKGKGITNASRVEHYLSDVCYTRAAELFKNAAIASGLRGKVKSNFRLKELKNMKSGLPTTKSDNFPIPLVKQKGGQHTGFEISSHNDDFIIKIPFGRWQVKKEIDKYRPWEKFDFEQVRKSPKPISLLLSTQRRKRNKGWSKDEGTEAEIRKVMNGDYQTSYIEVKRGSKTGEKSAWMLNLSIDVPKIDKGVDPSIIGGIDVGVKSPLVCAINNAFSRYSISDNDLFRFNKKMFARRRILLRKNRHKRAGHGAKNKLKPISILTGKSERFRKKLIERWACEIADFFIKNKVGTVQMENLESMKRKEDSYFNIRLRGFWPYAEMQNKIEFKLKQYGIVVRKVAPNNTSKTCSQCGHLNDYFNFEYRKKNKFPHFKCEKCNFKEDADYNAALNISNPKLKSTREEP

SEQ ID NO: 204 - protein, 726 aa, synthetic construct
SEVEFSHEYWMRRALTLAKRARDEREVPVGAVLVLNNRVIGVGWNRAVGLHDPTAHAEIMALRQGGLVMQNYRLTEATLYVTFEPCIMCAGAMIHSRIGRVVFGVRNSKRGAAGSLMNVLNYPGMNHRVEITEGILADECAALLCDYYRMPRQVFNARKKARSSINPGGSSGGSSGSETPGTSESPTPESPGGSSGGSAKNTITKTLKLRIVRPYNSAEVEKIVADEKNNRERIALEKNKDKVREACSKHLKVAAYCTTQVERNACLFCKARKLDDKFYQKLRGQFPDAVFWQEIGEIFRQLQKQAAEIYNQSLIELYYEIFIKGKGFANASSVEHYLSDVCYTRAAELFKNAAIASGLRGKVKSNFRLKELKNMKSGLPTTKSDNFPIPLVRQKGGQYTGFEISSHNDDLIIKIPFGRWQVKKEIDKYRPWEKFDFEQVRKSPKPISLLLSTRRRKRNKGWSKDEGTEAEIRKVMNGDYRTSYIEVKRGSKIGEKSAWMLNLSIDVPKIDKGVDPSIIGGIDVGVKSPLVCAINNAFSRYSISDNDLFRFNKKMFARRRILLGKNRHKRAGHGVKNKLKPITILTEKSGRFRKKLIERWACEIADFFIKNKVGTVQMEDLESMKRRGDSYFNIRLRGFWPYAEMQNKIEFKLKQYGIKIRKVAPNNTSKTCSKCGHLNNYFSFEYRKKNKFPHFKCEKCNFKEDADYNAALNISNPKLKSTKEEP

SEQ ID NO: 205 - protein, 726 aa, synthetic construct
SEVEFSHEYWMRHALTLAKRARDEREVPVGAVLVLNNRVIGEGWNRAIGLHDPTAHAEIMALRQGGLVMQNYRLTDATLYVTFEPCVMCAGAMIHSRIGRVVFGVRNSKRGAAGSLMNVLNYPGMNHCVEITEGILVDECAALLCDFYRMPRQVLNAQKKAQSSISSGGSSGGCSGSEMPGASESVTPKSSGGSSAGSTKNTITKTLKLRIVRPYNSAEVEKIVADEKNSREKIALERNKDKVKEACSEHLKVAAYCTTQVERNACLFCKARKLDDRFYQKLRGQFPDAVFWQETGEIFRQLQRQAAEIYNRSLIELYYEIFIKGKGFANASSVEHYLSDVCYTRAAELFKNAAIASGLRGKVKSNFRLKELKNMKSGLPTTKSDNFPIPLVKQKGGQYTGFEISSHNDDFIIKIPFGRWQVKKEIDKYRPWEKFDFEQVRKSPKPISLLLSTQRRKRNKGWSKDEGTEAEIRKVMNGDYQTSYIEVKRGSKIGEKSAWMLSLSIDVPKIDKGVDPSIIGGIDVGVKSPLVCAINNAFCRYSISDNDLFHFNKRMFARRRILLKKSRHKRAGHGAKNKLKPISILTEKSKRFRKKLIERWACEIADFFIKNKVGTVQMENLESMKRKEDSYFNIRLRGFWPYAEMQNKIEFKLKQYGIKIRKVAPNNTSRTCSKCGHLNNYFSFEYRKKNKFPHFKCEKCNFKEDADYNAALNISNPKLKGTKEEL

SEQ ID NO: 206 - protein, 726 aa, synthetic construct
SEVEFSHEYWMRHALTLAKRARDEREVPVGAVLVLNNRVIGVGWNRAIGLHDPTAHAEIMALRQGSLVMQNYRLTDATLYVTFEPCVMCAGAMVHSRIGRVVFGVRNSKRGAAGSLMNVLNYPGMNHCVEITEGILVDECAALLCDFYRMPRQVLNAQKKAQSSISSGGSSGGSSGSETPGTSESPTPESSGGSSGGPAKNTITKTLKLRIVRPYNSAEVEKIVADEKNNREKIALEKNKDKVKEACSKHLKVAAYCTTQVERNACLFCKARKLDDKFYQKLRGQFPDAVFWQELGEILRQLQKQAAEIYNQSLIELYYVIFIKGRGFANASSVEHYLSDVCYTRAAELFKNAAIASGLRGKVKSNFRLKELKNMKSGLPTTKSDNFPIPLVKQKGGQYTGFEISSHNDDFIIKIPFGRWQVKEEIDKYRPWEKFDFEQVRKNPKPISLLLSTQRRKRNKGWSKDEGTEAEIRKVMNGDYQTSYIEVKRGSKIGEKSAWMLNLSIDVPKIDKGVDPSIIGGIDVGVKSPLVCAINNAFSRYSISDNDLFRFNKKVFARRRILLKKNRHKRAGHGTKNKLKPITILTEKSGRFRKKLIERWACEIANFFIKNKVGTVQMENLESMKRKGDSYFNIRLRGFWPYAEMQNKIEFKLKQYGIKIRKVAPNNTSKTCSKCGHLNNYFSFEYRKKNKFPHFKCEKCNFKEDADYNAALNISNPKLKSTKEEP

SEQ ID NO: 207 - protein, 726 aa, synthetic construct
SEVEFSHEYWMRHALTLAKRARDEREVPVGAVLVLNNRVIGEGWNRAIGLHDPTAHAEIMALRQGGLVMQNYRLIDATLYVTFEPCVMCAGAMVHSRIGRVVFGVRNSKRGAAGSLMNVLDYPGMDHRVEITEGILADECAALLSDFYRMPRQVFNAQKKAQSSINSGGSSGGSSGSETPGTSESATPESSGGSSGGSAKNTITKTLQLRIVRPYNSAEVEKIVTDEKNNREKIALEKNKDKVKEACSKHLKMASYCTTQVERNACLFCKARKLDDKFYQKLRGQFPDAVFWQELGGIFRQLQKQAAEIYNQSLIELYYEIFIKGKGITNASRVEHYLSDVCYTRAAELFKNAAIASGLRSKVRSNFRLKELKNMKSGLPTTKSDNFPIPLVKQKGGQYTGFEISSHDDDFVIKIPFGRWQVKKEIDKYRPWEKFDFEQVRKSPKPISLLLSTQRRKRNKGWSKDEGTEAEIRKVMNGDYQTSYIEVKRGSKIGEKSAWMLNLSIDVPKIDKGVDPSIVGGIDVGVKSPLVCAINNSFSRYSICDNDLFRFNKKMFARRRILLKKNRHKRAGHGAKNKLKPITVLTKKSERFRKKLIERWVCEVADFFIKNKVGTVQMENLESMKRKEDSYFNIRLRGFWPYAEMQNRIELKLKQYGIEIRRVAPNNTSRTCSKCGHLNNYFNFEYRKKNKFPHFKCEKCNFREDADYNAALNISNPKLKSTKEEP

SEQ ID NO: 208 - protein, 726 aa, synthetic construct
GEVEFSHEYWMRRALTLAKRARDEREVPVGAILVLNNRVIGVGWNRAVGLHDPTAHAEIMALRQGGLVMQNYRLIEATLYVTFEPCIMCAGAMIHSRIGRVVFGVRNSKRGAAGSLMNVLNYPGMNHRVEITEGILADECAALLCDYYRMPRQVFNARKKAQPSTNSGGSSDGGSGSETPGTSESATPESSGGSSGGSAKNTITKTLKLRIVRPYNSAEVEKIVADEKSNREKIALEKNKDKVKEACSEHLKVASYCTTQVERNACLFCKARKLDDKFYQKLRGQFPDAVFWQELGEIFRQLQKQAAEIYNQSLIELYYEIFIKGKGFANASSVEHYLSDVCYTRAAELFKNAAIASGLRGKVKSNFRLKELKNMKSGLPTTKSDNFPIPLVKQKGGQYTGFEISNHNSDFIIKIPFGRWQVKKEINKYRPWEKFDFEQVRKSPKPISLLLSTQRRKRNKGWSKDEGTEAEIRKVMNGDYQTSYIEVKRGSKIGEKSAWMLNLSIDVPKIDKGVDPSIIGGIDVGVKSPLVCAINNAFSRYSISDNDLFHFNKKMFARRRILLKKNRHKRAGHGAKNKLKPITILTEKSRRFRKKLIERWACEIADFFIKNKVGTVQIENLESMKRKEDSYFNIRLRGFWPYAEMQNKIEFKLKQYGIEIRKVAPNNTSKTCSKCGHLNNYFNFEYRKKNKFPHFKCEKCNFREDADYNAALNISNPKLKSTKEEP

SEQ ID NO: 209 - protein, 726 aa, synthetic construct
SEVEFSHEYWMRHALTLAKRARDEREVPVGAVLVLNNRVIGEGWNRTIGLHDPTAHAEIMALRQGGLVMQNCRLTDATLYVTFEPCVMCAGAMIHSRIGRVVFGVRNSKRGAAGSLMNVLNYPGMNHCVEITEGILVDECAALLCDFYRMPRQVLNAQKKAQSSISSGGSSGGSSGSETPGAGESVTPKSSVGSSAGSTKNTITKTLKLRIVRPYNSAEVEKIVADEKNNREKIALEKNKDKVKEACSEHLKVAAYCTTQVERNACLFCKARKLDDKFYQKLRGQFPDAVFWQEIGEIFRQLQKQAAEVYNQSLIELYYEIFIKGKGIANASSVEHYLSDVCYTRAAELFKNAAIASGLRNKIKSNFRLKELRNMKSGLPTTKSDNFPIPLVKQKGGQYTGFEISSHNDDFIIKIPFGRWQVKKEIDKYRPWEKFDFEQVRKSPKPISLLLSTQRRRRNKGWSKDEGTEAEIRKVMYGDYQTSYIEVKRGSKIGEKSAWMLNLSIDVPKIDKGVDPSIIGGIDVGVKSPLVCAINNAFSRYSISDNDLFHFNKKMFARRRILLKKNRHKRAGHGARNKLKPITVLTEKSKRFRKKLIERWACEIANFFIKNKVGTVQMENLESMRRKEDSYFNIRLRGFWPYAEMQNKIEFKLKQYGIKIRKVAPNNTSKTCSKCGHLNNYFSFEYRKKNKFPHFKCEKCNFKENADYNAALNISNPKLRSTKEEP

SEQ ID NO: 210 - protein, 726 aa, synthetic construct
SEVEFSHEYWMRHALTLAKRARDEREVPVGAILVLNNRVIGEGWNRAIGLHDPTAHAEIMALRQGGLVMQNYRLIDATLYVTFEPCVMCAGAMIHSRIGRVVFGVRNNKHGAAGSLVNVLNYPGMNHRVEITEGILADECAALLCDFYRMPRQVFNARRKAQSSINPGGSSGGSSGSEAPGTSESATPESSGGSSGGSAKNTITKTLKLRIVRPYNSAEVEKIVADEKNSREKIALEKNKDKVKEACSKHLKVAAYCTTQVERNACLFCKARRLDDKFYQKLRGQFPDAVFWQEIGEIFRQLQKQAAEIYNQSLVELYYEILIKGKGIANASSVEHYLSDVCYTRAAELFKNAAIASGLRNKIKSNFRLKELRNMKSGLPTTKSDNFPIPLVRQKGGQYTGFEISNHDGDFIIKIPFGRWQVKKEINKHRPWEKFDFEQVRKSPKPISLLLSTQRRKRNKGWSKDEGTEAEIRKVMNGDYQTSYIEVKRGSKIGEKSAWMLSLSIDVPKIDKGVDPSIIGGIDVGVKSPLVCAINNAFSRYSISDNDLFRFNKKMFARRRILLKKNRHKRAGHGAKNKLKPITILTEKSKRFRRKLIERWACEIADFFIKNKVGTVQMENLESMKRKEDSYFNIRLRGFWPYAEMQDKIEFKLKQYGIKIRKVAPNNTSKTCSKCGHLNNYFNFEFRKKNKFPHFKCEKCNFKEDADYNAALNISNPKLKGTKEEP

SEQ ID NO: 211 - protein, 726 aa, synthetic construct
SEVEFSHEYWMRHALTLAKRARDEREVPVGAVLVLNNRVIGEGWNRAIGLHDPTAHAEIMALRQGGLVMQNYRLVDATLYVTFEPCVLCAGAMVHSRIGRVVFGVRNSKRGAAGSLMNVLNHPGMNHRVEITEGILADECAALLCDFYRMPRQVFNAQKKARSNINSGGSSGGSSGSETPGTSESATPVSSSGSSGGSAKNTITKTLKLRIVRPYNSAEVEKIVADEKNNREKIALEKNKDKVKEACSKHLKVAAYCTTQVERSACLFCRARRLDDKFYQKLRGQFPDAVFWQELGEIFRQLQKQAAEIYNQSLIELYYEIFIRGKGFANASSVEHYLSDVCYTRAAELFKNAAIASGLRGKVKSNFRLKELKNMKSGLPTTKSDNFPIPLVKQKGGQYTGFEISSHNDDFIIKIPFGRWQVKKEIDKYRPWEKFDFEQVRKSPKPISLLLSTQRRKRSKGWSKDEGTEAEIRKVMNGDYQTSYIEVKRGSKIGEKSAWMLNLSIDVPKIDKGVDPSIIGGIDVGVKSPLVCAINNAFSRYSVGDNDLFHYNKKMFARRRILLKKNRHKRAGHGAKNKLKPISILTEKSKRFRKKLIERWACEIADFFIKNKVGTVQIENLESMKRKEDSYFNIRLRGFWPYAEMQNKIEFKLKQYGIEIRKVAPNNTSKTCSKCGHLNSYFNFEYRKKNKFPHFKCEKCNFKEDADYNAALNISNPKLKSTKGEP

SEQ ID NO: 212 - protein, 726 aa, synthetic construct
SEVEFSHEYWMRHALTLAKRARDEREVPVGAILVLNNRVIGEGWNRAIGLHDPTAHAEIMALRQGGLVMQNYRLTDATLYVTFEPCVMCAGAMIHSRIGRVVFGVRNSKHGAAGSLMNVLNYPGMNHRVEITEGILADECAALLCDFYRMPRQVFNGRKKAQSGINSGGSSGGGSGSETPGTSESATPESSGGSFGGSAKNTITKTLQLRIVRPYNSAEVEKIVADEKNSREKIALEKNKDKVKEACGKHLKVASYCTTQVERNACLFCKARKLDDKFYQKLRGQFPDAVFWQELGEIFRQLQKQAAEIYNQSLIELYYEIFIKGKGLANASSVEHYLSDVCYTRAAELFKNAAIASGLRGKVKSNFKLKELKSMKSGLPSTKSDNFPIPLVKQKGGQYTGFEISSRNDDFIIKIPFGRWQVKKEIDKYRPWEKFDFEQVRKSPKPISLLLSTQRRKRNKGWSKDEGTEAEIRKVMNGDYQTSYIEVKRGRKIGEKSVWMLNLSIDVPKIDKGVDPSTIGGIDVGVKSPLVCAINNAFSRYSISDNDLFRFNKKMFARRRILLKKNRHKRAGHGAKNKLKPITILTEKSGRFRKKLIERWACEIADFFIRNKVGTVQMENLESMKRKEDSYFNIRLRGFWPYAEMQNKIELKLKQYGIKIRKVAPNNTSKTCSKCGHLNDYFNFEYRKKNKFPHFKCEKCNFKEDADYNAALNISNPKLKSTREEP

SEQ ID NO: 213 - protein, 726 aa, synthetic construct
SEVEFSHEYWMRHALTLAKRARDEREVPVGAVLVLNNRVIGVGWNRAIGLHDPTAHAEIMALRQGGLVMQNYRLTDATLYVTFEPCVMCAGAMVHSRIGRVVFGVRNSKRGAAGSLMNVLNYPGMNHRVEITEGILADECAALLCDFYRMPRQVFNARKKAQSSINPGGPSGGSSGSETPDTSESATPESSGGSSGSSAKNTITKTLQLRIVRPYNSAEVEKIVADEKNNREKIALEKNKDKVKEACSKHLKVAAYCTTQVERNACLFCKARRLDDKFYQKLRGQFPDAVFWQEIGEIFRQLQKQAAEIYNQSLIELYYEIFIKGKGFANASSVEHYLSDVCYTRAAELFKNAAIASGLRGKVKSNFKLKELKSMKSGLPSTKSDNFPIPLVKQKGGQYTGFEISSHNDDFVIKIPFGRWQVKKEIDRYRPWEKFDFEQVRKSPKPISLLLSTQRRKRNKGWSKDEGTEAEIRKVMNGDYQTSYIEVKRGSKIGEKSAWMLNLSIDVPKIDKGVDPSIIGGIDVGVKSPLVCAINNAFGRYSISDNDLFHFNKKMFARRRILLKKNRHKRAGHGAKNKLKPISILTEKSKRFRKKLIERWACEVADFFIKNKVGTVQMENLESMKRKEDSYFNIRLRGLWPYAEMQNKIEFKLKQYGIEIRKVAPNNTSKTCSKCGHLNNYFNFEYRKKNKFPHFKCEKCNFKENADYNAALNISNPKLKSTKEKP

SEQ ID NO: 214 - protein, 726 aa, synthetic construct
SEVEFSHEYWMRHALTLAKRARDEGEVPVGAVLVLNNRVIGEGWNRAIGLHDPTAHAEIMALRQGGLVMQNYRLVDATLYVTFEPCVLCAGAMVHSRIGRVVFGVRNSKRGAAGSLMNVLNYPGMNHRVEITEGILADECAALLCDFYRMPRQVFNARKKAQSSINPGGSSGGSSGSETPGTSESATPESSGGSSGSSAKNTITKTLKLRIVRPYNSAEVEKIVADEKNNREKIALEKNKDKVKEACSKHLKVAAYCTTQVERSACLFCKARRLDDKFYQKLRGRFPDAVFWQEIGEIFRQLQRQAAEVYNQSLVELYYEILIKGKGIANASSVEHYLSDVCYTRAAELFKNAAIASGLRNKIKSNFRLKELRNMRSGLPTTKSDNFPIPLVRQKGGQYTGFEISNHDGDFIIKIPFGRWQVKKEINKHRPWEKFDFEQVRKSPKPISLLLSTQRRKRNRGWSKDEGTEAEIRKVMNGDYQTSYIEVKRGSKIGEKSAWMLSLSIDVPKIDKGVDPSIIGGIDVGVKSPLVCAINNAFSRYSISDNDLFRFNKKMFARRRILLGKNRHKRAGHGVKNKLKPITILTEKSGRFRKKLIERWACEIADFFVKNKVGTVQMENLESMKRKEDSYFNIRLRGFWPYAEMQDKIEFKLKQYGIVVRKVAPNNTSKTCSKCGHLNHYFNFEYRKKNKFPHFKCEKCNFKEDADYNAALNISNPKLKSTKGEP

SEQ ID NO: 215 - protein, 726 aa, synthetic construct
SEVEFSHEYWMRHALTLAKRARDEREVPVGAVLVLNNRVIGEGWNRAIGLHDPTAHAEIMALRQGGLVMQNYRLIDATLYVTFEPCVMCAGAMIHSRIGRVVFGVRNNKHGAAGSLVNVLNYPGMNHRVEITEGILADECAALLCDFYRMPRQVFNARKKAQSSINPGGSSGGSSGSETPGTSESATPESSGGSSGGSAKSTITKTLKLRIVRPYNSAEVEKIVADEKNNREKIALEKNKGKVKEACSKHLKVAAYCTTQVERNACLFCKARRLDDKFYQKLRGQFPDAVFWQEIGEIFRQLQKQAAEVYNQSLIELYYEILIKGKGFANASSVEHYLSDVCYTRAAELFKNAAIASGLRGKVKSNFRLKELKNMRSGLPTTKSDNFPIPLVKQKGGQYTGFEISSHNSDFIIKIPFGRWRVKEEIDKYRPWEKFDFEQVRKSPKPISLLLSTQRRKKNKGWSKDEGTEAEIRRVMNGDYQTSYIEVKRGSKIGEKSAWMLNLSIDVPKIDKGVDPSIIGGIDVGVKSPLVCAINNSSSRYSICDNDLFRFNKKMFARRRILLKKNRHKRAGHGAKNKLKPITILTKKSERFRKKLIERWACEIADFFIKNKVGTVQMENLESMKRKEDSYFNIRLRGFWPYAEMQNKIEFKLKQYGIEIRKVAPNNTSKTCSKCGHLNNYFNFEYRKKNKFPHFKCEKCNFKENADYNAALNISNPKLKSTKETP

SEQ ID NO: 216 - protein, 726 aa, synthetic construct
SEVEFSHEYWMRRALTLAKRARDEREVPVGAVLVLNNRVIGVGWNRAIGLHDPTAHAEIMALRQGGLVMQNYRLTDATLYVTFEPCVMCAGAMIHSRIGRVVFGVRNNKHGAAGSLVNVLNYPGMNHRVEITEGILADECAALLCDFYRMPRQVFNARKKAQSSINPGGSSGGSSGSETPGTSESATPESSGGSSGSSAKNTITKTLKLRIVRPYNSAEVEKIVADEKNSREKIALEKNKDKVKEACSKHLKVAAYCTTQVERNACLFCKARKLDNKFYQKLRGQFPDAVFWQELGEIFRQLQKQAAEIYNQSLIELYYEIFIKGKGIANASRVEHYLSNVCYTRAAELFKNAAIASGLRSKVKSNFRLKELKSMKSGLPTTKSDNFPIPLVKQKGGQYTGFEISSHNDDFIIKIPFGRWQVKKEIDKYRPWEKFDFEQVRKSPRPISLLLSTQRRKRNKGWSKDEGTEAEIKKVMNGDYRTSYIEVKRGSKIGEKSAWMLNLSIDVPKIDKGVDPSIIGGIDVGVKSPLVCAINNAFSRYSISDNDLFRFNKKMFARRRILLEKNRHKRAGHGVKNKLKPITILTEKSRRFRKKLIERWACEIADFFIKNKVGTVQMENLESMKRKEDSYFNIRLRGFWPYAEMQNKIEFKLKQYGIKIRKVAPNNTSRTCSKCGHLNNYFSFEYRKKNKFPHFKCEKCNFKEDADYNAALNISNPKLKGTKEEL

SEQ ID NO: 217 - protein, 726 aa, synthetic construct
SEVEFSHEYWMRRALTLAKRARDGREVPVGAVLVLNNRVIGEGWNRAIGLHDPTAHAEIMALRQGGLVMQNYRLIDATLYVTFEPCVMCAGAMVHSRIGRVVFGVRNSKRGAAGSLMNVLDHPGMGHRVEITEGILADECAALLCDFYCMPRQVFNAQKRAQSSINSGGSSGGSSGSGTPGTSESATPESSGGGSSGSAKNTITKTLQLRIVRPYNSAEVEKIVADEKNNREKIALEKNKDKVKEACSKHLKVASYCTTQVERNACPFCKARKLDDKFYQKLRGQFPDAVFWQELGGIFRQLQKQAAEIYNQSLIELYYEIFIKGKGITNASRVEHYLSDVCYTRAAELFKNAAIASGLRSKVRSNFRLKELKNMKSGLPTTKSDNFPIPLVKQKGGQYTGFEISSHNSDFIIKIPFGRWQVKEEIDKYRPWEKFDFEQVRKSPKPISLLLSTQRRKRNKGWSKDEGTEAEIRKVMNGDYQTSYIEVKRGSKIGEKSAWMLNLSIDVPKIDKGVDPSIIGGIDVGVKSPLVCAINNTFSRYSISDNDLFRFNKKMFARRRILLGKNRHKRAGHGVKNKLKPITILTEKSGRFRKKLIERWACEIADFFVKNKVGTVQMENLESMKRKEDSYFNIRLRGFWPYAEMQNKIEFKLKQYGIEIRKVAPNNTSKTCSKCGHLNNYFNFEYRKKNKFPHFKCEKCNFKENADYNAALNISNPKLKSTKEEP

SEQ ID NO: 218 - protein, 726 aa, synthetic construct
SEVEFSHEYWMRHALALAKRARDEREVPVGAVLVLNNRAIGEGWNRAIGLHDPTAHAEIMALRQGGLVMQNYRLTDATLYVTFEPCVMCAGAMIHSRIGRVVFGVRNSKRGAAGSLMNVLNYPGMNHCVEITEGILVDECAALLCDFYRMPRQVLNAQKKAQSSISSGGSSGGSSGSETPGASGSVTPKSSGGSSAGSTKDTITKTLKLRIVRPYNSAEVEKAVADEKNNREKIAIEKNKDKVKEACSKHLKVAAYCTTQVERNACLFCRARRLDDKFYQKLRGQFPDAVFWQELGEIFRQLQKQAAEIYNQSLIELYYEIFIKGKGFANASSVEHFLSDVCYTRAAELFKNAAIASGLRNKIKSNFRLKELRNMKSGLPTTKSDNFPIPLVRQKGGQYTGFEISSHNSDFIIKIPFGRWQVKKEIDKYRPWEKFDFEQVRKSPKPISLLLSTQRRKRNRGWGKDEGTEAEIKRVMNGDYQTSYIEVKRGSKIGEKSAWMLNLSIDVPKIDKGVDPRIIGGIDVGVKSPLVCAINNAFSRYSISDNDLFHFNKKMFARRRILLKKNRHKRAGHGTKNKLKPISILTEKSKRFRKKLIERWACEIADFFIKNKVGTVQMENLESMKRKEDSYFNIRLRGFWPYAEMQNKIEFKLKQYGIEIRKVAPNNTSKTCSKCGHLNNYFNFEYRRKNKFPHFKCEKCNFKEDADYNAALNISNPKLKSTKEGP

SEQ ID NO: 219 - protein, 726 aa, synthetic construct
SEVEFSHEYWMRHALTLAKRARDEREVPVGAVLVLNNRVIGEGWNRAVGLHDPTAHAEIMALRQGGLVMQNYRLTDATLYVTFEPCVMCAGAMIHSRIGRVVFGVRNSKRGAAGSLMNVLNYPGMNHCVEITEGILVDECAALLCDFYRMPRRVLNAQKKAQSSISSDGSSGGSSCSETPGASESVTPKSSGGSSGGSAKNTITKTLKLRIVRPYNSAEVEKIVADEKNNRERIALEKNKDKVKEACSKHLKVATYCTTQVERNACLFCKARRLDDKFYQKLRGQFPDAVFWQELGEIFRQLQKQAAEIYNQSLIELYYEIFIKGKGLANASSVEHYLSDVCYTRAAGLFKNAAIASGLRGKVKSNFKLKELKSMKSGLPSTKSDNFPIPLVKQKGGQYTGFEISSHNDDLIIKIPFGRWQVKKEIDKYRPWEKFDFEQVRKSPKPISLLLSTQRRKRNKGWSKDEGTEAEIRKVMNGDYQTSYIEVKRGSKIGEKSAWMLNLSIEVPKIDKGVDPCIIGGIDVGVKSPLVCAINNAFSRYSISDNDLFHFNKKMFARRRILLKKNGHKRAGHGAKNKLKPITIMTEKSKRFRKKLIERWACEIANFFIKNKVGTVQMENLESMKRREDSYFNIRLRGFWPYAEMQSKIEFKLKQYGIEVRKVAPNNTSKTCSKCGHLNNYFNFEFRKKNKFPHFKCEKCNFKEDADYNAALNISNPKLKSTKEVP

SEQ ID NO: 220 - protein, 726 aa, synthetic construct
SEVEFSHEYWMRHALSLAKRARDEREVPVGAVLVLNNRIIGEGWNRAIGLHDPTAHAEIMALRQGGLVMQNYRLTDATLYVTFEPCVMCAGAMVHSRIGRVVFGVRNSKRGAAGSLMNVLNYPGVNHCVEITEGILVDECAALLCDFYRMPRQVLNAQKKAQSSISPGGSSGGCSGSEMPGASESVTPKSSGGSSAGSTKNTITKTLKLRIVRPYNSAEVEKIVADEKNSREKIALERNKDKVKEACSEHLKVAAYCTTQVERNACPFCKARKLDDRFYQKLRGQFPDAVFWQETGEIFRQLQRQAAEIYNQSLIELYYEIFIKGKGFANASSVEHYLSDVCYTRAAELFKNAAIASGLRGKIKSNFRLKELKNMKSGLPTTKSDNFPIPLVKQKGGQYTGFEISNHNSDFIIKIPFGRWQVKKEIDKYRPWEKFDFEQVRKSPKPISLLLSTQRRKRNKGWSKDEGTEAEIKRVMNGDYQISYIEVKRGSKIGEKSAWMLSLSVDVPKIDKGVDPSIIGGIDVGVKSPLVCAINNAFSRYSISDNDLFHFNKKMFARRRILLKKSKHKRAGHGAKNKLKPITILTEKSKRFRKKLIERWACEIADFFIKNKVGTVQMENLESMKKKEDSYYNIRLRGFWPYAEMQNKIEFKLKQYGIEIRKVAPNNTSRTCSKCGHLNNYFNFEYRKKNKFPHFKCEKCNFKEDADYNAALNISNPKLKSTREEP

SEQ ID NO: 221 - protein, 726 aa, synthetic construct
NEVEFSHEYWMRHALTLAKRARDGREVPVGAVLVLNNRVIGEGWNRAIGLHDPTAHAEIMALRQGGLVMQNYRLIDATLYVTFEPCVMCAGAMVHSRIGRVVFGVRNSKRGAAGSLLNVLDHPGMDHRVEITEGILADECATLLCDFYRMPRQVFNAQKKAQSSINSGGSSGGSSGSETPGTSESATPESSGGSSGGSAKNTITKTLQLRIVRPYNSAEVEKIVADEKNNREKVALEKNKDKVKEACSEHLKVAAYCTTQVERSACLFCKARKLDDKFYQKLRGQFPDAVFWQEIGEIFRQLQKQAAEIYNQSLIELYYEIFIKGRGFANASSVEHYLSDVCYTRAAELFKNAAIASGLRGKVKSNFRLKELKNMKSGLPTTKSDNFPIPLVKQKGGQYTGFEISSHNDDFIIKIPFGRWQVKKEIDKYRPWEKFDFAQVRRSPKPISLLLSTQRRKRNKGWSKDEGTEAEIRKVMNGDYQTSYIEVKRGSKIGEKSAWMLNLSIDVPRIDKGVDPSIIGGIDVGVKSPLVCAINNALSRYSISDNDLFHFNKKMFARRRILLRKNRHKRAGHGAKNKLKPITIMTEKSKRFRKKLIERWACEIADFFIKNKVGTVQMENLESMKRKEDSYFNIRLRGFWPYAEMQNKIEFKLKQYGIVVRKVAPNNTSKTCSKCGHLNNHFNFEYRKKNKFPHFKCEKCNFKEDADYNAALNISNPKLKSTKGEP

SEQ ID NO: 222 - protein, 726 aa, synthetic construct
SEVEFSHEYWMRHALSLAKRARDEREVPVGAVLVLNNRIIGEGWNRAIGLHDPTAHAEIMALRQGGLVMQNYRLTDATLYVTFEPCVMCAGAMVHSRIGRVVFGVRNSKRGAAGSLMNVLNYPGMNHCVEITEGILADECAALLCDFYRMPRQVFSARKKAQSSINSGGSSGGNSGSKTPGTSESATPESSGGSSGGSAKNTITKTLKLRIVRPYNSAEVEKIVADEKNDREKIALEKNKDKVKEACSKHLKVAAYCTTQVERNACQFCKARKLDDKFYQKLRGQFPDAVFWQEIGEIFRQLQKQAAEIYNQSLVELYYEILIKGKGIANASSVEHYLSDVCYTRAAELFKNAAIASGLRGKVKSNFRLKELKNMKSGLPTTKSDNFPIPLVKQKGGQYTGFEISSHNDDFIIKIPFGRWQMKKEIDRYRPWEKFDFEQVRKSPKPISLLLSTQRRKRNKGWSRDEGTEAEIRKVMNGDYQTSYIEVKRGSKIGEKSAWMLSLSIDVPKIDKGVDPSIIGGIDVGVKSPLVCAINNAFSRYSISDNDLFRFNKKMFARRRILLKKSRHKRAGHGAKNKLKPISILTEKSKRFRKKLIERWACEIADFFIKNKVGTVQMENLESMKRKEDSYFNIRLRGFWPYAEMQNKIEFKLKQYGIEIRKVAPNNTSKTCSKCGHLNNYFNFEYRKKNKFPHFKCERCNFKENADYNAALNISNPKLKSTKEEP

SEQ ID NO: 223 - protein, 726 aa, synthetic construct
SEVEFSHEYWMRHALTLAKRARDEREVPVGAVLVLNNRVIGEGWNRTTGLHDPTAHAEIMALRQGGLVMRNYRLTDATLYVTFEPCVMCAGAMIHSRIGRVVFGVRNSKRGAAGSLMNVLNYPGMNHCVEITEGILVDECAALLCDFYRMPRQVLNAQKKAQSSISPGGSSGGSSGSETPGASESVTPKSSGGSSGGSAKNTITKTLKLRIVRPYNSAEVEKIVADEKNNREKIALEKNKGKVKEACSRHLEVAAYCTTQVERNACLFCKARKLDDKFYQKLRGQFPDAVFWQELGEIFRQLQKQAAEIYNQSLIELYYEIFIKGKGFANASSVEHYLSDVCYTRAAELFKNAAIASGLRGKVKSNFRLKELKNMRSGLPTTKSDNFPIPLVKQKGGQYTGFEISSHNDDFIIKIPFGRWQAKKEIDKYRPWEKFDFEQVRKSPKPISLLLSTQRRKRNRGWSKDEGTEAEIRKVMNGDYQTSYIEVKRGSKIGEKSAWMLNLSIDVPKIDRGVDPSIIGGIDVGVKSPLVCAINDAFSRYSISDNDLFRFNKKMFARRRILLGKNRHKRAGHGVKNKLKPITILTEKSGRFRKKLIERWACEIADFFVKNKVGTVQMENLESMKRKEDSYFNIRLRGFWPYAEMQNKIEFKLKQYGIKVRKVAPNNTSKTCSKCGHLNNYFNFEYRKKNKFPHFECEKCNFKENADYNAALNICNPKLKSTKGEP

SEQ ID NO: 224 - protein, 726 aa, synthetic construct
SEVEFSHEYWMRHALTLAKRARDEREVPVGAVLVLNNRVIGEGWNRAIGLNDPTAHAEIMALRQGGLVMQNYRLIDATLYVTFEPCVMCAGAMIHSRIGRVVFGVRNNKHGAAGSLVNVLNYPGMNHRVEITEGILADECAALLCDFYRMPRQVFNARKKAQSSINPGGSSGGSGGSETPGTSESATPESSGGSSGSSAKNTITKTLKLRIVRPYNSAEVEKIVADEKNNREKIALEKNKDKVKEACSEHLKVAAYCTTQVERSACLFCKARKLDDKFYQKLRGQFPDAVFWQEIGEIFRQLQKQAAEIYNQSLIELYYQIFIKGKGFANASSVEHYLSDVCYTRAAELFKNAAIASGLRGKVKSNFRLKELKNMKSGLPTTKSDNFPIPLVRQKGGQYTGFEISSHNDDFIIKIPFGRWQVKKEIDKYRPWEKFDFEQVRKSPKPISLLLSTRRRKRNKGWSKDEGTEAEIRKVMNGDYQTSYIEVKRGSKTGEKSAWMLNLSIDVPKIDKGVDPSIIGGIDVGVKSPLVCAINNAFGRYSISDNDLFHFNKKMFARRRILLKKNRHKRAGHGAKNKLKPITILTEKSKRFRKKLIERWACEIADFFIKNKVGTVQMENLESMKRKEDSYFNVRLRGFWPYAEMQNKIEFKLKQYGIEIRKVAPNNTSKTCSKCGHLNNYFNFEYRRKNKFPHFKCEKCNFKEDADYNAALNISNPKLKSTKEEP

SEQ ID NO: 225 - protein, 726 aa, synthetic construct
SEVEFSHEYWMRHALSLAKRARDEREVPVGAVLVLNNRIIGEGWNRAIGQHDPTAHAEIMALRQGGLVMQNNRLTDATLYVTFEPCVMCAGAMVHSRIGRVVFGVRNSKRGAAGSLMNVLNYPGVNHCVEITEGILVDECAALLCDFYRMPRQVLNAQKKAQSSISPGGSSGGSSGSETPGASESVTPKSSGGSSGGSAKNTITKTLKLRIVRPYNSAEVEKIVADEKNNREKIALEKNKGKVKEACSKHLEVAAYCTTQVERNACLFCKARKLDDKFYQKLRGQFPDAVFWQEIGEIFRQLQKQAAEIYNQSLIELYYEIFIKGKGITNASRVEHYLSDVCYTRAAELFKNAAIASGLRSKVRSNFRLKELKNMKSGLPTTKSDNFPIPLVKQKGGQYTGFEISSHNDDFIIKIPFGRWQVKKEIDKYRPWEKFDFEQVRKSPKPISLLLSTQRRRRSKGWSKDEGTEAEIRKVMNGDYQTSYIEVKRGSKIGEKSAWMLSLSIDVPKIDKGVDPSIIGGIDVGVKSPLVCAINNAFCRYSISDNDLFHFNKKMFARRRILLKKNRRKRDGHGAKNKLKPITILTEKSKRFRKKLIERWACEIADFFIKNKVGTVQMENLESMKRKEDSYFNIRLRGFWPYAEMQDKIEFKLKQYGIEIRKVAPNNTSKTCSRCGHLNNYFNFEYRRKNKFPHFKCEKCNFKEDADYNAALNISNPKLKSTKEEP

SEQ ID NO: 226 - protein, 726 aa, synthetic construct
SEVEFSHEYWMRHALTLAKRARDEREVPVGAILVLNNRVIGEGWNRAIGLHDPTAHAEIMALRQGGLVMQNYRLIDATLYVTFEPCVMCAGAMIHSRIGRVVFGVRNNKHGAAGSLVNVLDYPGMNHRVEITEGILADECAALLCDFYRMPRQVFNARKKAQSSISPGGSSGGSSGSETPGAIESVTPKSSGGRSGGSAKNTFTKTLKLRIVRPYNSAEVEKIVADEKNNREKIALEKNKGKVKEACSKHLEVAAYCTTQVERSACLFCKARKLDDKFYQKLRGQFPDAVFWQELGEIFRQLQKQAAEIYNQSLIELYYEIFIKGKGFANASSVEHYLSDVCYTRAAELFKNAAIASGLRGKVKSNFRLKELKNMKSGLPTTKSDNFPIPLVKQKGGQYTGFEISSHNDDFIIKIPFGRWQVKEEIDKYRPWEKFDFEQVRKNPKPISLLLSTQRRKRNKGWSKDEGTEAEIRKVMNGDYQTSYIEVKRGSKIGEKSAWMLNLSIDVPKIDKGVDPSIIGGIDVGVKSPLVCAINNAFSRYSIGDNDLFHYNKKMFARRRILLKKNRHKRAGHGAKNKLKPISILTEKSKRFRKKLIERWACEIADFFIKNKVGTVQIENLESMKRKEDSYFNIRLRGFWPYAEMQNKIEFKLKQYGIEIRKVAPNNTSKTCSKCGHLNSYFNFEYRKKNKFPHFKCEKCNFKEDADYNAALNISNPKLKSTKEEP

SEQ ID NO: 227 - protein, 726 aa, synthetic construct
SEVEFSHEYWMRHALTLAKRARDEREVPVGAVLVLNNRVIGEGWNRAIGLHDPTAHAEVMALRQGGLVMQNYRLTDATLYVTFEPCVMCAGAMIHSRIGRVVFGVRNSKHGAAGSLVNVLNYPGMNHRIEITEGILADECAALLCDFYRMPRQVFNARKKAQSSINSGGSSGGSSGSETPGTSESATPKNSGGSSGGSAKNTITKALKLKIVRPYNSAEVEKIVADEKNNRERIALEKNKDKVKEACSKHLKVAAYCTTQVERNACLFCKARKLDDKFYQKLRGQFPDAVFWQEIGEIFRQLQKQAAEIYNQSLIELYYEIFIKGKGFANASSVEHYLSDVCYTRAAELFKNAAIASGLRGKVKSNFRLKELKNMKSGLPTTKSDNFPIPLVKQKGGQYTGFEISDHNGDFIIKIPFGRWQVKKETNKYRPWEKFDFEQVRKSPKPISLLLSTQRRKRNKGWSKDEGTEAEIRKVMNGDYQTSYIEVKRGSKIGEKSAWMLNLSIDVPKIDKGVDPSIIGGIDVGVKSPLVCAINNALSRYSISDNDLFHFNKKMFARRRILLKKTRHKRAGHGAKNKLKPISILTEKSERFRKKLIERWACEIADFFIKNKVGTVQMENLESMKRREDSYFNIRLRGFWPYAKMQNKIEFKLKQYGIEIRKVAPNNTSKTCSKCGHLNNYFNFEYRKKNKFPHFKCERCNFKENADYNAALNISNPKLKSTKEEP

SEQ ID NO: 228 - protein, 726 aa, synthetic construct
SEVEFSHEHWMRHALTLAKRARDEREVPVGAVLVLNNRVIGEGWNRTTGLHDPTAHAEIMALRQGGLVMQNHRLVDATLYVTFEPCVMCAGAMIHSRIGRVVFGVRNSKHGAAGSLVNVLNYPGMNHRVEITEGILADECAALLCDFYRMPRQVFNTRKKAQSSINPSGSSGGSSGSVTPGTSESATPESSGGGFGGSAKNTITKTLKLRIVRPYNSAEVEKIVADEKNSREKIALERNKDKVKEACSEHLKVAAYCTTQVERNACLFCKARKLDDRFYQKLRGQFPDAVFWQETGEIFRQLQKQAAEIYNQSLIELYYEIFIKGKGFANASSVEHYLSDVCYTRAAELFKNAAIASGLRGKVKSNFRLKELKNMKSGLPTTKSDNFPIPLVKQKGGQYTGFEISNHNGDFIIKIPFGRWQVKKEINKYRPWEKFDFEQVRKSPKPISLLLSTQRRKRNKGWSKDEGTEAEIKKVMNGDYQISYIEVKRGSKIGEKSAWTLNLSVDVPKIDKGVDPSIIGGIDVGVKSPLVCAINNALSRYSISDNDLFHFNKKVFARRRILLKKNRHRRAGHGAKNKLKPITILTEKSKRFRKKLIERWACEIADFFIKNKVGIVQMENLESMKRREDSYFNIRLRGFWPYAEMQNKIEFKLKQYGIGIRKVAPNNTSKTCSRCGHLNNYFNFEHRKKNKFPRFKCEKCNFKENADYNAALNISNPKLKSTKEEP

SEQ ID NO: 229 - protein, 726 aa, synthetic construct
SEVEFSHEYWMRHALTLAKRARDEREVPVGAVLVLNNRVIGEGWNRTTGLHDPTAHAEIMALRQGGLVMQNHRLVDATLYVTFEPCVMCAGAMIHSRIGRVVFGVRNSKRGAAGSLTNVLNYPGMNHRVEITEGILVDECAALLCDFYRMPRQVFNAQKKAQSSINSGGSSGGNSGSKTPGTSESAAPESFGGSSGGSAKNTITKTLKLRIVRPYNSAEVEKIVADEKNNREKIALEKNKDKVKEACSKHLKVAAYCTTQVERNACLFCKARKLDDKFYQKLRGQFPDAVFWQEISEILRQLQKQAAEIYNRSLVELYYEIFIKGKGIANASRVEHYLSDVCYTRAAELFKNAAIASGLRGKVKSNFRLKELKNMKSGLPTTKSDNFPIPLVKQKGGQYTGFEVSSHNDDFIIKIPFGRWQVKKEIDKYRPWEKFDFEQVRKSPKPISLLLGTQRRKRNKGWGKDEGTEAEIRKVMNGDYQTSYIEVKRGSKIGEKGAWMLSLSIDVPKIDKGVDPRIIGGIDVGVKSPLVCAINNAFSRYSISDNDLFRFNKKMFARRRILLKKNRHKRAGHGAKNKLKPITILTEKSVRFRKKLIERWACEIADFFIKNKVGTVQMENLESMKGKEDSYFNVRLRGFWPYAEMQNKIEFKLKQYGIEIRKVAPNNTSKTCSKCGHLNNYFNFEYRKKNKFPHFKCEKCYFKEDADYNAALNISNPRLKSTKEEP

SEQ ID NO: 230 - protein, 726 aa, synthetic construct
SEVEFSHEYWMRHALTLAKRARDEREVPVGAVLVLNNRVIGEGWNRAIGLHDPTAHAEIMALRQGGLVMQNYRLIDATLYVTFEPCVMCAGAMIHSRIGRVVFGVRNSKRGAAGSLTNVLNYPGMNHRVEITEGILVDECAALLCDFYRMPRQVFNAQKKAQSSISSGGPSGGSSCSETPGASESVTPKSSGGSSTGSTKDTITKTLKLRIVRPYNSAEVEKIVADEKNSREKIALEKNEGKVKEACSKHLKVATYCTTQVERSACLFCKARKLDDKFYQKLRGQFPDAVFWQEIGEIFRQLQKQAAEIYNQSLIELYYEIFIKGKGIASASRVGHYLSDVCYTRAAELFKNAAIASGLRGKVKSNFRLKELKNMRSGLPTTKSDNFPIPLVKQKGGQYTGFEISSHNDDFIIKIPFGRWQVKKEIDKYRPWEKFDFEQVRKSPKPISLLLSTQRRKRNKGWSKDEGTEAEIRKVMNGDYQTSYIEVKRGSKTGEKSAWMLNLSIDVPKIDKGVDPSIIGGIDVGVKSPLVCAINNAFSRYSISDNDLFRFNKKMFARRRILLKKNRHKRAGHGAKNKLKPITIMTEKSKRFRKKLIERWACEIADFFIKNKVGTVQMENLESMKRKEDSYFNIRLRGFWPYAEMQNKIEFKLKQYGIETRKVAPNNTSKTCSKCGHLNNYFNFEYRKKNKFPHFKCEKCNFKEDADYNAALNISNPQLKSTKGEP

SEQ ID NO: 231 - protein, 726 aa, synthetic construct
SEVEFSHEYWMRHALTLAKRARDEREVPVGAILVLNNRVIGEGWNRAIGLHDPTAHAEIMALRQGGLVMQNYRLIDATLYVTFEPCVMCAGAMIHSRIGRVVFGVRNNKHGAAGSLVNVLDYPGMNHRVEITEGILADECAALLCDFYRMPRQVFNARKKAQSSISPGGSSGGSSGSEAPGTSESATPESSGGSSGGSAKNTITKTLKLRIVRPYNSAEVEKIVADEKNNREKIALEKNKDKVKEACSEHLKVAAYCTTQVERSACLFCKARTLDDKFYQKLRGQFPDAVFWQEIGEIFRQLQKQAAEIYNQSLIELYYEIFIKGKGFANASSVEHYLSDVCYTRAAELFKNAAIASGLRGKVKSNFRLKELKNMKSGLPTTKSDNFPIPLVKQKGGQYTGFEISSHNGDFIIKIPFGRWQVKKEIDKYRPWEKFDFEQVRKSPKPISLLLSTQRRKRNKGWSKDEGTEAEIRKVMNGDYQTSYIEVKRGSKTGEKSAWMLNLSIDVPKIDKGVDPSIIGGIDVGVKSPLVCAINSAFSRYSISDNDLFRFNKKMFARRRILLKKNRHKRAGHGVKNKLKPISILTEKSKRFRKKLIERWACEIADFFIKNKVGTVQMENLEGMKRKEDSYFNIRLRGFWPYAEMQNKIEFKLKQYGIEIRKVAPNNTSKTCSKCGHLNNYFNFEYRRKNKFPHFKCEKCNFKEDADYNAALNISNPKLKSTKEEP

SEQ ID NO: 232 - protein, 726 aa, synthetic construct
SEVEFSHEYWMRHALTLAKRARDEREVPVGAILVLNNRVIGEGWNCAIGLHDPTAHAEIMALRQGGLVMQNYRLIDATLYVTFEPCVMCAGAMIHSRIGRVVFGVRNSKRGAAGSLMNVLNYPGMNHRVEITEGILVDECAALLCDFYRMPRRVLNAQKKAQSSISSGGSSGGSGGGETPGASESVTPKNSGGSSAGSTKNTITKTLKLRIVRPYNSAEVEKIVADEKNSREKIALEKNKGKVKEACREHLKVASYCTTLVERNACPFCKARKLDDKFYQKLRGQFPDAVFWQELGEILRQLQKQAAEIYNQSLIELYYEIFIKGRGFANASSVEHYLSDVCYTRAADLFKNAAIASGLRGKVKGNFRLKELRNMKSGLPTTKSDNFPIPLVKQKGGQYTGFEISSHNDDFIIKIPFGRWQVKKEIDKYRPWERFDFEQVRKSPKPISLLLSTQRRKRNKGWSKDEGTEAEIRKVMNGDYQTSYIEVKRGSKTGEKSTWMLNLSIDVPKIDKGVDPSIVGGIDVGVKSPLVCAINNAFSRYSISDNDLFRFNKKMFARRRVLLKKNRHKRAGHGAKNKLKPISILTEKSVRFRKKLIERWACEIADFFIKNKVGTVQMENLESMKGKEDSYFNIRLRGFWPYAEMQNKIEFKLKQYGIGIRKVAPNNTSKTCSKCGHLNNYFSFEYRKKNKFPHFKCEKCNFKENADYNAALNISNPKLKSTKEEP

SEQ ID NO: 233 - protein, 726 aa, synthetic construct
SEVEFSHEYWMRHALTLAKRARDEREVPVGAILVLNNRVIGEGWNRAIGLHDPTAHAEIMALRQGGLVMQNYRLIDATLYVTFEPCVMCAGAMVHSRIGRVVFGVRNSKHGAAGSLVNVLNYPGMNHRVEITEGILADECAALLCDFYRMPHQVFNARKKAQSSINPSGSSGGSSGSETPGTGGSATPEGSGSSSGGFAKSTITKTLKLRIVRPYNSAEVEKIVADEKDNREKIALEKNKGKVKEACSKHLKVAAYCTTQVERNACLFCKARRLDDKFYQKLRGQFPDAVFWQEIGEIFRQLQKQAAEIYNQSLIELYYEIFIKGKGFANASSVEHYLSDVCYTRAAELFKNAAIASGLRGKVKSNFRLKELKNMKSGLPTTKSDNFPIPLVKQKGGQYTGFEISSHNDDFIIKIPFGRWQVKKEIDKYRPWEKFDFEQVRKSPKPISLLLSTQRRKRNKGWGKDEGTEAEIRKVMNGDYRTSYIEVKRGSKIGEKSAWMLSLSIDVPKIDKGVDPRIIGGIDVGVKSPLVCAINDAFSRYSISDNDLFHFNKKMFARRRILLKRNRHRRAGHGVKNKLKPITILTEKSGRFRKKLIERWACEIADFFVKNKVGTVQMENLESMKRKEDSYFNIRLRGFWPYAEMQNKIEFKLKQYGIKVRKVAPNNTSKTCSKCGHLNNYFSFEYRKKNKFPHFKCEKCNFKENADYNAALNISNPKLKSTKEKP

SEQ ID NO: 234 - protein, 726 aa, synthetic construct
SEVEFSHEYWMRHALTLAKRARDEREVPVGAVLVLNNRVIGEGWNRAIGLHDPTAHAEIMALRQGGLVMQNYRLIDATLYVTFEPCVMCAGAMIHSRIGRVVFGVRNNKHGAAGSLVNVLDYPGMNHRVEITEGILADECAALLCDFYRMPRQVFNARKKAQSSISPGGSSGGSSGSETPGTNESATPESSGGSSGGSAKNTITKTLKLRIVRPYNSAEVEKIVADEKNNREKIALEKNKDKVKEACSKHLKMASYCTTQVERNACLFCKARKLDDKFYQKLRGQFPDAVFWQELGGIFRQLQKQAAEIYNQSLIELYYEIFIKGKGITNAGRVEHYLSDVCYTRAAELFKNAAIASGLRSKVRSNFRLKELKSMKSGLPTTKSDNFPIPLVKQKGGQYTGFEISSHNSDFIIKIPFGRWQVKEEIDKYRPWEKFDFEQVRKSPKPISLLLSTQRRKKNKGWSKDEGTEAEIRRVMNGDYQTSYIEVKRGSKIGEKSAWMLNLSIDVPKIDKGVDPSIIGGIDVGVKSPLVCAINNAFSRYSISDNDLFRFNKKVFARRRILLKKNRHKRAGHGAKNKLKPISILTGKSERFRKKLIERWACEIADFFIKNKVGTVQMENLESMKRKEDSYFNIRLRGFWPYAEMQNRIEFKLKQYGIEIRKVAPNNTSKTCSKCGHLNNYFNFEYRKKNKFPHFRCEKCNFKENADYNAALNISNPKLKSTKEEP

SEQ ID NO: 235 - protein, 726 aa, synthetic construct
SEVEFSHEYWMRHALALAKRARDEREVPVGAILVLNNRVIGEGWNRAIGLHDPTAHAEIMALRQGGLVMQNYRLIDATLYVTFEPCVMCAGAMIHSRIGRVVFGARNNKHGAAGSLVNVLNYPGMNHRVEITEGILADECAALLCDFYRMPRQVFNARKKAQSSINPGGSSGGSSGSETLGTREGATPESSGGSSGGSAKNTITKTLKLRIVRPYNSAEVEKIVADEKNNREKIALEKNKDKVKEACSKHLKVASYCTTQVERNACPFCKARKLDDKFYQKLRGQFPDAVFWQELGEILRQLQKQAAEIYNQSLIELYYEIFIKGRGFANASSVEHYLSDVCYTRAAELFKNAAIASGLRGKVKSNFRLKELKNMKSGLPTTKSDNFPIPLVRQKGGQYTGFEISSHNDDFIIKIPFGRWQVRKEIDKYRPWEKFNFEQVRKSPKPISLLLSTQRRKRNKGWSKDEGTEAEIRKVMNGDYQTSYIEVKRGSKIGEKSAWMLNLSIDVPKIDKGVDPSIIGGIDVGVKSPLVCAINNVLSRYSISDNDLFHFNKKMFARRRILLKKNGHKRAGHGTKNKLKPITILTEKSGRFRKKLIERWACEIANFFIKNKVGTVQMENLEGMKRKEDSYFNIRLRGFWPYAEMQNKIEFKLKQYGIKIRKVAPNNTSKTCSKCGHLNNYFSFEYRKKNKFPHFKCEKCNFKEDADYNAALNISNPKLKGTKEEP

SEQ ID NO: 236 - protein, 726 aa, synthetic construct
SEVEFSHEYWMRHALTLAKRARDEREVPVGAVLVLNNRVIGEGWNRAIGLHDPTAHAEIMALRQGGLVMQNHRLIDATLYVTFEPCVMCAGAMIHSRIGRVVFGVRNNKRGAAGSLMNILNYPGMNHRVEITEGILADECAALLCDFYRMPRQVFNAQKKARSNINSGSSSGGSSGSETPGTSESATPESSGGGSGGSAKNTITKALKLRIVRPYNSAEVEKIVADEKNSREKIALEKNKDKVREACSKHLKVASYCTTQVERYACPFCKARKLDDKFYQKLRGQFPDAVFWQELGEILRQLQKQAAEIYNQSLIELYYEIFIKGKGFANASSVEHYLSDVCYTRAAELFKNAAIASGLRGKVKSNFRLKELKNMKSGLPTTKSDNFPIPLVKQKGGQYTGFEISDHNSDFIIKIPFGRWQVKEEIVKYRPWEKFDFEQVRKSPKPISLLLSTQRRKRNKGWSKDEGTEAEIRKVMNGDYQTSYIEVKRGSRIGEKSAWMLSLSIDVPKIDKGVDPSIIGGIDVGVKSPLVCAINNAFGRYSISDNDLFHFNKKMFARRRILLKRNRHKRAGHGAKNKLKPITILTEKSKRFRKKLIERWACEIAGFFIKNKVGTVQMENLESMKRKEDSYFNIRLRGFWPYAEMQNKIEFKLKQYGIEVRKVAPNNTSKTCSKCGHLNNYFNFEYRRKNKFPHFKCEKCNFKEDADYNAALNISNPKLKSTKEEP

SEQ ID NO: 237 - protein, 726 aa, synthetic construct
SEVEFSHEYWMRHALSLAKRARDEREVPVGAVLVLNNRIIGEGWNRAIGLHDPTAHAEIMALRQGGLVMQNYRLTDATLYVTFEPCVMCAGAMVHSRIGRVVFGVRNSKRGAAGSLMNVLNYPGVNHCVEITEGILVDECAALLCDFYRMPRQVLNAQKKAQSSISSGGSSGGCSGSEMPGASESVTPKSSGGSSAGSTKNTITKTLQLRIVRPYNSAEVEKIVADEKNSREKIALERNKDKVKEACSKHLKVASYCTTQVERNACLFCKARKLDDKFYQKLRGQFPDAVFWQELGEIFRQLQKQAAEIYNQSLIELYYEIFIKGKGLANASSVEHYLSDVCYTRAAELFKNAAIASGLRGKVKSNFKLKELKSMKSGLPSTKSDNFPIPLVKQKGGRYTGFEISSHNDDLIIKIPFGRWQVKKEIDKYRPWEKFDFERVRKSPKPISLLLSTQRRKGNKGWSKDEGTEAEIRKVMNGDYQTSYIEVKRGSKIGEKSAWMLNLSIDVPKIDKGVDPSIIGGIDVGVKSPLVCAINDAFSRYSISDNDLFRFNKKMFARRRILLRKNRHKRAGHGAKNKLKPISILTERSERFRKKLIERWACEIADFFIKNKVGTVQMENLESMKRKEDSYFNIKLRGFWPYAEMQNKIEFKLKQYGIEIRKVAPNNTSKTCSKCGHLNNYFSFEYRKKNKFPHFKCEKCNFKENADYNAALNISNPKLKSTKEEP

SEQ ID NO: 238 - protein, 726 aa, synthetic construct
SEVEFSHEYWMRHALTLAKRARDEREVPVGAVLVLNNRVIGEGWNRAIGLHDPTAHAEIMALRQGGLALQNYRLVDATLYVTFEPCVLCAGAMVHSRIGRVVFGARNSKRGAAGSLMNILNYPGMNHRVEITEGILADECAALLCDFYRMPRQVFNAQEKAQSSISPGGSSGGSSGSETPGASESVTPKSSGGSSGGSAKNTITKTLKLRIVRPYNSAEVEKIVADEKNNREKIALEKNRGKVKEACSKHLEVAAYCTTQVERNACLFCKARKLDDKFYQKLRGQFPDAVFWQELGEIFRQLQKQAAEIYNQSLIELYYEIFIKGKGFANASSVEHYLSDVCYTRAAELFKNAAIASGLRGKVKSNFRLKELKNMKSGLPTTKSDNFPVPLVKQKGGQYTGFEISSHNDDFIIKIPFGRWQVRKEIDKYRPWEKFNFEQVRKSPKPISLLLSTQRRKRNKGWSKDEGTEAEIKKVMNGDYQTSYIEVKRGGKIGEKSAWMLSLSIDVPKIDKGVDPSIIGGIDVGVKSPLVCAINNAFSRYSISDNDLFRFNKKMFARRRILLGKNRHKRAGHGVKNKLKPITILTEKSGRFRKKLIERWACEIADFFVKNKVGTVQMENLESMRRKEDSYFNIRLRGFWPYAEMQNKIEFKLKQYGIKVRKVAPNNTSKTCSKCGHLNNYFSFEYRKKNKFPHFKCEKCNFKENADYNAALNISNPKLKSTKEEP

SEQ ID NO: 239 - protein, 726 aa, synthetic construct
SEVEFSHEYWMRHALTLAKRARDEREVPVGAVLVLNNRVIGEGWNRAIGLHDPTAHAEIMALRQGGLVMQNYRLSDATLYVTFEPCVMCAGAMIHSRIGRVVFGVRNSKRGAAGSLMNVLNYPGMNHCVEITEGILVDECAALLCDFYRMPRQVLSAQKKAQSSVSSGDSSGGSSGSETPGASGSVTPKSSVGSSAGSTKNTITKALKLRIVRPYNSAEVEKIVADEKNNREKIALEKNKDKVKEACSKHLKVAAYCTTQVERNACLFCKARKLDDKFYQKLRGQFPDAVFWQETGEIFRQLQRQAAEIYNQSLIELYYEIFIKGKGFANASSVEHYLSDVCYTRAAELFKNAAIASGLRGKVKGNFRLKELKNMKSGLPTTKSDNFPIPLVKQKGGQYTGFEISSHNDDFIIKIPFGRWQAKKEIDKYRPWEKFDFEQVRKSPKPISLLLSTQRRKRNKGWSKDEGTEAEIRRVMNGDYQTSYIEVKRGSKIGEKSAWMLNLSIDVPKIDKGVDPSIIGGIDVGVKSPLVCAISNAFSRYSISDNDLFHFNKKMFARRRILLKKSKHKRAGHGAKNKLKPITILTEKSRRFRKKLIERWACEIADFFIKNKVGTVQMENLESMKRREDSYFNIRLRGFWPYAEMQNKIEFKLKQYGIEIRKVAPNNTSKTCSKCGHLNNYFNFEYRKKNKFPHFKCERCNFKENADYNAALNISNPKLKSTKEEP

SEQ ID NO: 240 - protein, 726 aa, synthetic construct
SEVEFSHEYWMRHALTLAKRARDEREVPVGAVLVLNNRVIGEGWNRAIGLHDPTAHAEIMALRQGGLVMQNYRLIDATLYVTFEPCVMCAGAMIHSRIGRVVFGVRNNKRGAAGSLMNVLNYPGMNHRVEITEGILADECAALLCDFYCMPRQVLNAQKKARSCINSGGSSGGSSGSETPGTSESATPESSGGSSGGSAKNTITKTLKLRIVRPYNSAEVEKIVADEKNNREKIALEKNKDKVREACSKHLKVASYCTTQVERNACPFCKARKLDDKFYQKLRGQFPDAVFWQELGEILRQLQKQAAEIYNQSLIELYYEIFIKGRGFANASSVEHYLSDVCYTRAADLFRNAAIASGLRGKVKGNFRLKELKNMKSGLPTTKSDNFPIPLVKQKGGQYTGFEISSHDDDFIIKIPFGRWQVKKEIDKYRPWEKFDFEQVRKSPKPISLLLSTQRRKRNKGWSKDEGTEAEIRKVMNGDYQTSYIEVKRGSKTGEKSAWMLNLSIDVPKIDKGVDPSIIGGIDVGVKSPLVCAINNAFSRYSISDNDLFHFNKKMFARRRILLRKNGHKRAGHGAKNKLKPLTILTGKSKRFRKKLIERWACEIADFFIKNKVGTVQMENLESMKRKEDSYFNIRLRGFWPYAEMQNKIEFKLKQYGIKIRKVAPNNTSKTCSKCGHLNNYFNFEYRKKNKFPHFKCEKCNFKENADYNAALNISNPKLKSTKEEP

SEQ ID NO: 241 - protein, 726 aa, synthetic construct
SEVEFSHEYWMRHALTLAKRARDEREVPVGAVLVLNNRVIGEGWNRATGQNDPTAHAEIMALRQGGLVMQNHRLIDATLYVTFEPCVMCAGAMIHSRIGRVVIGVRNSRRGAAGSLMNVLNHPGMNHRVEITEGILADECAALLCDFYRMPRQVFNAQEKAQSSTNSGGSSGGSSGSETPGTSESVTPESSGGGSSGSAKNTITKTLQLRIVRPYNSAEVEKIVADEKNNREKIALEKNKDKVREACNKHLKVASYCTTQVERNACPFCKARKLDDKFYQKLRGQFPDAVFWQELGEILRQLQKQAAEIYNQSLIELYYEIFIKGKGFANASSVEHYLSDVCYTRAAELFKNAAIASGLRNKIKSNFRLKELRNMKSGLPTTKSDNFPIPLVRQKGGQYTGFEISNHNDDFIIKIPFGRWQVKKEIDKYRPWEKFDFEQVRKSPKPISLLLSTQRRKRNKGWNKDEGTEAEIRKVMNGDYQTSYIEVKRGSRIGEKSAWMLNLSIDVPKIDKGVDPSIIGGIDVGVKSPLVCAINNALSRYSISDNDLFHFNKKMFARRRILLKKNGHKRAGHGAKNKLKPITIMTEKSKRFRKKLIERWACEIADFFIKNKVGTVQMENLESMKRKEDSYFNIRLRGFWPYAEMQNKIEFKLKQYGIKIRKVAPNNTSRTCSKCGHLNNYFSFEYRKKNKFPHFKCEKCNFKEDADYNAALNISNPKLKGTKEEL

SEQ ID NO: 242 - protein, 726 aa, synthetic construct
SEVEFSHEYWMRHALTLARRARDEREVPVGAILVLNNRVIGEGWNRAIGLHDPTAHAEIMALRQGGLVMQNYRLIDATLYVTFEPCAMCAGAMIHGRIGRVVFGVRNNKHGAAGSLMNVLNYPGMDHRVEITEGILADECAALLCDFYRMPRQVFNARKKAQSSTNSGGSSDGGSGSETPGTSESATPENSGGSSGGSAKNTITKTLKLRIVRPYNSAEVEKIVADEKNNREKIALEKNKDKVKEACSEHLKVAAYCTTQVERSACLFCKARKLDDKFYQKLRGQFPDAVFWQEIGEIFRQLQKQAAEIYNQSLIELYYEIFIKGKGFANASSVEHYLSDVCYTRAAELFKNAAIASGLRGKVKSNFRLKELKNMRSGLPTTKSDNFPIPLVKQKGGQYTGFEISSHNDDFIIKIPFGRWQVKKEIDKYRPWEKFDFEQVRKSPKPISLLLSTQRRKRNKGWSKDEGTEAEIRKVMNGDYQTSYIEVKRGSKTGEKSTWMLNLSIDVPKIDKGVDPSIIGGIDVGVKSPLVCAINNAFSRYSISDNDLFRFNKKMFARRRILLKKNRHKRAGHGAKNKLKPISILTGKSERFRKKLIERWACEIADFFIKNKVGTVQMENLESMKRKEDSYFNIRLRGFWPYAEMQNKIEFKLKQYGIEIRKVAPNNTSKTCSKCGHLNYYFNFEYRKKNKFPHFKCEKCNFKENADYNAALNISNPKLKSTKEKP

SEQ ID NO: 243 - protein, 726 aa, synthetic construct
SEVELSHEYWMRHALTLAKRARDEHEVPVGAVLVLNNRVIGEGWNRAIGLHDPTAHAEIMALRQGGLVMQNYRLTDATLYVTFEPCVMCAGAMIHSRIGRVVFGVRNSKRGAAGSLMNVLNYPGMNHCVEITEGILVDECAALLCDFYRMPRQVLNAQKKAQSSISSGGSSGGSSGSETSGASGSVTPKSSGGSSGGSAKNTITKTLKLRIVRPYNSAEVEKIVADEKNNREKIALEKNKGKVKEACSKHLEVAAYCTTQVERNACLFCKARKLDDKFYQKLRGQFPDAVFWQELGEIFRQLQKQAAEIYNQSLIELYYEIFIKGKGFANASSVEHYLSDVCYTRAAELFKNAAIASGLRGKVKSNFRLKELKNMRGGLPTTKSDNFPIPLVKQKGGQYTGFEISSHNDDFIIKIPFGRWQVKKEIDKYRPWEKFDFEQVRKSPKPISLLLSTRRRKGNKGWSKDEGTEAEIRRVMNGDYQTSYIEVKRGSKIGEKSAWMLSLSIDVPKIDKGVDPRIIGGIDVGVKSPLVCAINNVLSRYSISDNDLFHFNKKMFARRRILLKKNGHKRAGHGAKNKLKPITIMTEKSKRFRKKLIERWACEIADFFIKNKVGTVQMENLESMKRKEDSYFNIRLRGFWPYAEMQNKIEFKLKQYGIVVRKVAPDNTSKTCSQCGHLNNYFNFEYRKKNQFPYFKCEKCNFKENADYNAALNISNPQLKSTKGEP

SEQ ID NO: 244 - protein, 726 aa, synthetic construct
SEVEFSHEYWMRHALTLAKRARDEREVPVGAVLVLNNRVIGEGWNRAIGLHDPTAHAEIMALRQGGLVMQNYRLIDATLYVTFEPCVMCAGAMIHSRIGRVVFGVRNSKHGAAGSLVNVLNYPGMNHRVEITEGILADECAALLCDFYRMPRQVFNARKKAQSSINPSGSSGGSSGNVTPGTSESATPESSGGGFGGSAKNTITKTLQLRIVRPYNSAEVEKIVADEKNNREKIALEKNKDKVKEACSKHLKVASYCTTQVERNACLFCKARKLDDKFYQKLRGQFPDAVFWQELGEIFRQLQKQAAEIYNQSLIELYYEIFIKGKGIANASSVGHYLSDVCYTRAAELFKNAAIASGLRGKVKSNFRLKELKNMKSGLPTTKSDNFPIPLVKQKGGQYTGFEISSHNDDFIIKIPFGRWQVRKEIDKYRPWEKFNFEQVRKSPKPISLLLSTQRRKRNKGWSMDEGTEAEIRKVMNGDYQTSYIEVKRGRKIGERSAWMLNLSIDVPKIDKGVDPNTIGGIDVGVKSPLVCAINNAFSRYSISDNDLFHFNKKMFARRRILLKKNRHKRAGHGAKNKLKPITILTEKSKRFRKKLIERWASEIADFFIKNKVGTVQMENLESMKRKEDSYFNIRLRGFWPYAEMQNKIEFKLKQYGIEVRKVAPNNTSKTCSKCGHLNNYFDFEYRKKNKFPHFRCEKCNFKENADYNAALNISNPKLKSTKEEP

SEQ ID NO: 245 - protein, 726 aa, synthetic construct
SEVEFSHEYWMRHALTLAKRARDEREVPVGAVLVLNNRVIGEGWNRAIGLHDPTAHAEIMALRQGGLVMQNYRLSDATLYVTFEPCVMCAGAMIHSRIGRVVFGVRNSKRGAAGSLMNVLNYPGMNHCVEITEGILVDECAALLCDFYRMPRQVLSAQKKAQSSISSGGSSGGSSGSETPGASGSVTPKSSGGGFGNSAKNTITKTLKLRIVRPYNSAEVEKIVADEKNNREKIALEKNKDKVQEACSKHLKVASYCTTQVERNACLFCKARKLDDKFYQKLRGQFPDAVFWQELGEIFRQLQKQAAEIYNQSLIELYYKIFIKGKGLANASNVEHYLSDVCYTRAAELFKNAAIASGLRGKVKSNFKLKELKSMKSGLPSTKSDNFPIPLVKQKGGQYTGFEISSHNDDFIIKIPFGRWQVKEEIDKYRPWEKFDFEQVRKSPKPISLLLSTQRRKRNKGWSKDEGTEAEIRKVMNGDYQTSYIEVKRGSKIGEKSAWMLNLSIDVPMIDKGVDPSIIGGIDVGVKSPLVCAINNAFSRYSIGDNDLFHYNKKMFARRRILLKKNRHKRAGHGAKNKLKPISILTEKSKRFRKKLIERWACEIADFFIKNKVGTVQIENLESMKRKEDSYFNIRLRGFWPYAEMQNRIEFKLKQYGIEIRKVAPNNTSKTCSKCGHLNSYFNFEYRKKNKFPHFKCEKCNFKENADYNAALNISNPKLKSTKGEP

SEQ ID NO: 246 - protein, 726 aa, synthetic construct
SEVEFSHEYWMRHALTLAKRARDEREVPVGAVLVLNNRVIGEGWNRAIGLHDPTAHAEIMALRQGGLVMQNYRLVDATLYVTFEPCVLCAGAMVHSRIGRVVFGVRNSKRGAAGSLMNVLNYPGMNHRVEITEGILVDECAALLCDFYRMPRQVLNAQKKAQSSISSGGSSGGSSGSVTPGASGSVTPKSSGGSSAGSTKDTITKTLKLRIVRPYNSAEVEKIVADEKNNREKIALEKNKGKVKEACSKHLKVATYCTTQVERNACLFCKARKLDDKFYQKLRGQFPDAVFWQEVGEIFRQLQKQAAEIYNQSLIELYYEIFIKGKGIANASSVGHYLSDVCYTRAAELFKNAAIASGLRGKIKSNFRLKELKNMKSGLPTTKSDNFPIPLVKQKGGQYTGFEISNHNGDFIIKIPFGRWQVKKEINKYRPWEKFDFEQVRKSPKPISLLLSTQRRKRNKGWSKDEGTEAEIRRVMNGDYQTSYIEVKRGSKIGEKSAWMLNLSIDVPKIDKGVDPSIIGGIDVGVKSPLVCAINNSSSRYSICDNDLFRFNKKMFARRRILLKKNRHKRAGHGAKNKLKPITIMTEKSKRFRKKLIERWACEIADFFIKNKVGTVQIEDLESMKRKEDSYFNIRLRGFWPYAEMQNKIEFKLKQYGIKIRRVAPNNTSKTCSKCGHLNNYFNFEYRRKNKFPHFKCEKCNFKEDADYNAALNISNPKLKSTKEEP

SEQ ID NO: 247 - protein, 726 aa, synthetic construct
SEVEFSHEYWMRHALTLAKRARDEREVPVGAVLVLNNRVIGEGWNRAIGLHDPTAHAEIMALRQGGLVMQNYRLTDATLYVTFEPCVMCAGAMVHSRIGRVVFGVRNSKRGAAGSLMNVLNYPDMNHCVEITEGILVDECAALLCDFYRMPRQVLNSQKKAQSSISSGGSSGGSSGSETPGASESATPKSSGGSSAGSTKDTITKTLKLRIVRPYNSAEVEKIVADEKNSREKIALEKYKDKVKEACSEHLKVAAYCTTQVERNACLFCKARKLDDRFYQKLRGQFPDAVFWQELGEILRQLQKQAAEIYNQSLIELYYEIFIKGKGFANASSVEHYLSDVCYTRAAELFKNAAIASGLRGKVKSNFRLKELKNMRSGLPTTKSDNFPIPLVKQKGGQYTGFEISSHNDDFIIKIPFGRWQVKKEIDRYRPWERFDFEQVRKSPKPISLLLSTQRRKRNKGWSKDEGTEAEIRKVMNGDYQTSYIEVKRGSKIGEKSAWMLNLSIDVPKIDKGVDPSIIGGIDVGVKSPLVCAINNAFSRYSISDNDLFRFNKKMFARRRILLKKNRHKRAGHGAKNKLKPVSILTEKSERFRKKLIERWACEIADFFIKNKVGTVQMENLESMKRREDSYFNIRLRGFWPYAEMQNKIEFKLKQYGIEIRKVAPNNTSKICSKCGHLNNYFNFEYRRKNKFPHFKCEKCNFKENADYNAALNISNPKLKSTKEEP

SEQ ID NO: 248 - protein, 726 aa, synthetic construct
SEVEFSHEYWMRHALTLAKRARDEREVPVGAILVLNNRVIGEGWNRAIGLHDPTAHAEIMALRQGGLVMQNYRLIDATLYVTFEPCVMCAGAMIHSRIGRVVFGVRNSKHGAAGSLVNVLNYPGMNHRVEITEGILADECAALLCDFYRMPRQVFNARKKAQSSINPSGSSGGSSGSVTPGTSESATPESSGGGFGGSVKNTITKTLQLRIVRPYNSAEVEKIVADEKNNREKIALEKNKDKVKEACSKHLKVASYCTTQVERNACLFCKARKLDDKFYQKLRGQFPDAVFWQEIGEIFRQLQKQAAEIYNQSLIELYYEIFIKGKGFANASSVEHYLSDVCYTRAAELFKNAAIASGLRGKVKSNFRLKELKNMKSGLPTTKSDNFPIPLVKQKGGQYTGFEISSHNDDFIIKIPFGRWQVKEEIDKYRPWEKFDFEQVRKSPKPISLLLSTQRRKRNKGWSKDEGTEAEIRKVMNGDYQTSYIEVKRGRKIGEKSVWMLNLSIDVPKIDEGVDPSTIGGIDVGVKSPLVCAINNAFSRYSISDNDLFRFNKKMFARRRILLKKNRHKRAGHGAKNKLKPITILTEKSGRFRKKLIERWACEIADFFIKNKVGTVQMENLGSMKRKEDSYFNIRLRGFWPYAEMQNKIELKLKQYGIKIRKVAPNNTSKTCSKCGHLNDYFNFEYRKKNKFPHFKCEKCNFKEDADYNAALNISNPKLKSTKGEP

SEQ ID NO: 249 - protein, 726 aa, synthetic construct
SEVEFSHEYWMRHALTLAKRARDEREVPVGAVLVLNNRVIGEGWNRAIGLHDPTAHAEIMALRQGGLAMQNYRLVDATLYVTFEPCVLCAGAMVHSRIGRVVFGVRNSKRGAAGSLMNVLNHPGMNHRVEITGGILADECAALLCDFYRMPRQAFNAQKKAQSSISPGGSSGGSSGSETPGTSESATPKNSGGSSGGSAKNTITKALKLKIVRPYNSAEVEKIVADEKNNRERIALEKNKDKVKEACCEHLKVATYCTTQVERNACLFCKARKLDDKFYQKLRGQFPDAVFWQEIGEIFRQLQKQAAEIYNQSLIELYYEIFIKGKGITNASRVEHYLSDVCYTRAAELFKNAAIASGLRSKVRSNFRLKELKNMKSGLPTTKSDNFPIPLVKQKGGQYTGFEISSHNDDFIIKIPFGRWQAKKEIDKYRPWEKFDFEQVRKSPKPISLLLSTQRRKRNKGWSKDEGTEAEIRKVMNGDYQTSYIEVKRGSKTGEKSAWMLNLSIDVPKIDKGVDPSIIGGIDVGVKSPLVCAINNAFSRYSISDNDLFRFNKKMFARRRILLKKNRHKRAGHGAKNKLKPISILTGKGERFRKKLIERWACEIADFFIKNKVGTVQMENLESMKRKEDSYFNIRLRGFWPYAEMQNKIEFKLKQYGIEIRKVAPNNTSKTCSKCGHLNNYFNFEYRKKNKFPHFKCEKCNFKENADYNAALNISNPKLKSTKEEP

SEQ ID NO: 250 - protein, 726 aa, synthetic construct
SEVEFSHEYWMRRALTLAKRARDEREVPVGAVLVLNNRVIGVGWNRAVGLHDPTAHAEIMALRQGGLVMQNYRLIDATLYVTFEPCVMCAGAMIHSRIGRVVFGVRNSKHGAAGSLVNVLNYPGMNHRVEITEGILADECAALLCDFYRMPRQVFNARKKAQSSVNSGGSSGGSSGSETPGTSESATPKSSGGSSGGSAKNTITKALKLRIVRPYNSAEVEKIVADEKNNREKIALEKNKDKVKEACSKHLKMASYCTTQVERNACLFCKARKLDDKFYQKLRGQFPDAVFWQEIGEIFRQLQRQAAEIYNQSLIELYYEIFIKGKGFANASSVEHYLSDVCYTRAAELFKNAAIASGLRGKVKSNFRLKELKNMKSGLPTTKSDNFPIPLVKQKGGQYTGFEISSHNDDFIIKIPFGRWQVKKEIDKYRPWEKFDFEQVRKSPKPISLLLSTQRRKRNKGWSKDEGTEAEIRKVMNGDYQTSYIEVKRGRKIGEKSAWMLNLSIDVPKIDKGVDPSIVGGIDVGVKSPLVCAIDNALSRYSISDNDLFHFNKKMFARRRILLKKNRHRRAGHGAKNKLKPISILTEKSKRFRKKLIERWASEIADFFIKNKVGTVQMENLESMKRKEDSYFNIRLRGFWPYAEMQNKIEFKLKQYGIEIRKVAPNNTSKTCSKCGHLNNYFNFEYRKKNKFPHFKCEKCNFKENADYNAALNISNPKLKSTKEEP

SEQ ID NO: 251 - protein, 726 aa, synthetic construct
GEVEFSHEYWMRHALTLAKRARDEREVPVGAILVLNNRVIGEGWNRAIGLHDPTAHAEIMALRQGGLVMQNYRLIDATLYVTFEPCVMCAGAMIHSRIGRVVFGVRNSKHGAAGSLVNILNYPGMNHRVEITEGILVDECAALLCDFYRMPRQVLNAQKKAQSSISSGGSSGGCSGSEMPGTSESATPESSGGSSGGSAKNTITKTLQLRIVRPYNSAEVEKIVTDEKNNREKIALEKNKDKVKEACSKHLKMASYCTTQVERNACLFCKARKLDDKFYQKLRGQFPDAVFWQELGVIFRQLQKQAAEIYNQSLIELYYEIFIKGKGITNASRVEHYLSDVCYTRAAELFKNAAIASGLRSKVRSNFRLKELKNMKSGLPTTKSDNFPIPLVKQKGGQYTGFEISSHNDDFIIKIPFGRWQVKKEINKYRPWEKFDFEQVRKSPKPISLLLSTQRRKRNKGWSKDEGTEAEIRKVMNGDYQTSYIEVKRGSKTGEKSAWMLNLSIDVPKIDKGVDPSIIGGIDVGVKSPLVCAINNAFSRYSISDNDLFRFNKKMFARRRILLKKNRHKRAGHGAKNKLKPISILTERSERFRKKLIERWACEIADFFIKNKVGTVQMENLESMKRKEDSYFNIRLRGFWPYAEMQNKIEFKLKQYGIEIRKVAPNNTSKTCSKCGHLNNYFNFEYRKRNKFPHFKCEKCNFKENADYNAALNISNPKLKSTKEEP

SEQ ID NO: 252 - protein, 726 aa, synthetic construct
SEVEFSHEYWMRHALTLAKRARDEREVPVGAVLVLNNRVIGEGWNRAIGLHDPTAHAEIMALRQGGLVMQNYRLTDATLYVTFEPCVMCAGAMIHSRIGRVVFGVRNSKRGAAGSLTNVLNYPGMNHRVEITEGILVDECAALLCDFYRMPRQVFNARKKAQSSINPGGSSGGSSGSETPGTSESATPESSGGSSAGSTKDTITKTLKLRIVRPYNSAEVEKIVADEKNSREKIALEKNKDKVKEACSEHLKVAAYCTTQVERNACPFCKARKLDDKFYQKLRGQFPDAVFWQEVGEIFRQLQKQAAEIYNQSLIELYYEIFIKGKGFANASSVEHYLSDVCYTRAAELFKNAAIASGLRGKVKSNFRLRELKSMKSGLPTTKSDNFPIPLVKQKGGQYTGFEISNHNSDFIIKIPFGRWQVKKEINKYRPWEKFDFEQVRKSPKPISLLLSTQRRKRNKGWSKDEGTEAEIRKVMNGDYQISYIEVKRGSRIGEKSAWMLNLSIDVPKIDKGADPSIIGGIDVGVKSPLVCAINNAFSRYSISDNDLFRFNKKMFARRRILLKKNRHKRAGHGIKNKLKPIAILTEKSGRFRKKLIERWACEIANFFIKNKVGTVQMENLESMKRKEDSYFNIRLRGFWPYAEMQNKIEFKLKQYGIKIRKVAPNNTSKTCGKCGHLNNYFSFEYRKKNKFPHFKCEKCNFKEDADYNAALNISNPKLKSTKEEP

SEQ ID NO: 253 - protein, 726 aa, synthetic construct
SEVEFSHEYWMRHALTLAKRARDEREVPVGAVLVLNNRVIGEGWNRAIGLHDPTAHAEIMALRQGGLVMQNYRLSDATLYVTFEPCVMCAGAMIHSRIGRVVFGVRNSKRGAAGSLMNVLNYPGMNHCVEITEGILVDECAALLCDFYRMPRQVLSAQKKAQSSISSGGSSGGSSGSETPGASGSVTPKSSVGSSAGSTKNTITKTLKLRIVRPYNSAEVEKIVADEKNNREKIALEKNKDKVKEACSEHLKVAAYCTTQVERNACLFCKARRLDDKFYQKLRGQFPDAVFWQEIGEIFRQLQKQAAEIYNQSLVELYYEIFIKGKGIANASSVEHYLSDVCYTRAAELFKNAAIASGLRSKVRSNFRLKELKNMKSGLPTTKSDNFPIPLVRQKGGQYTGFEISNHNGDFIIKIPFGRWQVKKEINKHRPWEKFDFEQVRKSPKPISLLLSTQRRKRNKGWGKDEGTEAEIRKVMNGDYQTSYIEVKRGSKIGEKSAWMLNLSIDVPKIDKGVDPSIIGGIDVGVKSPLVCAINNAFSRYSISDNDLFRFNKKMFARRRILLRKNRHKRAGHGAKNKLKPISVLTGKSERFRKKLIERWACEIADFFIKNKVGTVQMENLESMKRKEDSYFNIRLRGFWPYAEMQNKIELKLKQYGIEIRKVAPNNTSKTCSKCGHLNDYFNFEYRKKNKFPHFKCEKCNFKEHADYNAALNISNPKLKSTKEEP

SEQ ID NO: 254 - protein, 726 aa, synthetic construct
SEVEFSHEYWMRHALTLAKRARDEREVPVGAILVLNNRVIGVGWNRAIGLHDPTAHAEVMALRQGGLVTQNYRLIDATLYVTFEPCVMCAGAMIHSRIGRVVFGVRNSKHGAAGSLVNVLNYPGMNHRVEITEGILADECAALLCDFYRMPRQVFNARKKAQSSINSGGSSGGSSGSETPGTSESATPKSSGGSSGGSAKNTITKALKLRIVRPYNSAEVEKIVADEKNNRERIALEKNKDKVKEACSKHLKVAAYCTTQVERNACLFCKARKLDDKFYQKLRGQFPDAVFWQEIGEIFRQLQKQAAEIYNQSLIELYYEIFIKGKGFANASSVEHYLSDVCYTRAAELFKNAAIASGLRGKVKSNFRLKELKNMRSGLPTTKSDNFPIPLVKQKGGQYAGFEISSHNDDFIIKIPFGRWQVKKEIDKYRPWEKFDFEQVRKSPKPISLLLSTRRRKRNKGWSKDEGTEAEIRKVMNGDYQISYIEVKRGSKIGEKSAWMLNLSIDVPKIDKGVDPSIIGGIDVGVKSPLVCAINNAFGRYSISDNDLFRFNKKVFARRRILLKKNRHKRAGHGTKNKLKPITILTEKSGRFRKKLIERWACEIANFFIKNKVGTVQMENLESMKRKEDSYFNIRLRGFWPYAEMQNKIEFKLKQYGIKIRKVAPNNTSKTCSKCGHLNNYFGFEYRKKNKFPHFKCEKCNFKEDADYNAALNISNPKLKSTKEEP

SEQ ID NO: 255 - protein, 726 aa, synthetic construct
SEVEFSHEYWMRHALSLAKRARDEREVPVGAVLVLNNRIIGEGWNRAIGLHDPTAHAEIMALRQGGLMMQNHRLIDATLYVTFEPCVLCAGAMVHSRIGRVVFGVRNSKRGAAGSLMNVLNYPGMNHRVEITEGVLADECAALLCDFYRMPRQVFNAQKKAQSSINSGGSSGGSSGSETSGTSESPTPESSGGSSGGSAKNTITKTLKLRIVRPYNSAEVEKIVADEKNNREKIALEKNKDKVKEACSKHLEVAAYCTTQVERNACLFCKARKLDDKFYQKLRGQFPDAVFWQELGEIFRQLQKQAAEIYNQSLIELYYEIFIKGKGSANASSVEHYLSDVCYTRAAGLFKNAAIASGLRGKVKSNFRLKELKNMKSGLPTTKSDNFPIPLVKQKGGQYTGFEISSHNDDFIIKIPFGRWQVKKEIDKYRPWEKFDFEQVRKSPKPISLLLSTQRRKRNKGWSKDEGTEAEIRKVMNGDYQTSYIEVKRGSKTGEKSAWMLSLSIDVPKIDKGVDPSIIGGIDVGVKSPLVCAINNAFSRYSISDNDLFRFNKKMFARRRILLKKNRHKRAGHGAKNKLKPISILTGKSGRFRKKLIERWACEIADFFVKNKVGTVQMENLESMKRKEDSYFNIRLRGFWPYAEMQNKIEFKLKQYGIVVRKVAPNNTSKTCSKCGHLNNYFSFEYRKKNKFPHFKCEKCNFKENADYNAALNISNPKLKSTKEEP

SEQ ID NO: 256 - protein, 726 aa, synthetic construct
SEVEFSHEYWMRHALTLAKRARDEREVPVGAVLVLNNRVIGEGWNRAIGLHDPTAHAEIMALRQGGLVMQNYRLTDATLYVTFEPCVMCAGAMIHSRIGRVVFGVRNSKRGAAGSLMNVLNYPGMNHCVEITEGILVDECAALLCDFYRMPRQVLNAQKKAQSSISSGGSSGGSSGSETPCASESVTPKSSGGSSAGSTKNTLTKTLKLRIVRPYNSAEVEKIVADEKNNREKIALEKNKGKVKEACSKHLEVAAYCTTQVERNACLFCKARKLDDKFYQKLRGQFPDAVFWQEIGEIFRQLQKQAAEIYNQCLIELYYEIFIKGKGFANASSVEHYLSDVCYTRAAELFKNAAIASGLRGKVKSNFRLKELKNMRSGLPTTKSDNFPIPLVKQKGGQYAGFEISSHNDDFIIKIPFGRWQVKKEIDKYRPWEKFDFEQVRKSPKPISLLLSTRRRKRNKGWSKDEGTEAEIRKVMNGDYQTSYIEVKRGSKIGEKSAWMLNLSIDVPKIDKGVDPSIIGGIDVGVKSPLVCAINNAFGRYSISDNDLFHFNKKMFARRRILLKKNRHKRAGHGARNKLKPITILTEKSKRFRRKLIERWACEIADFFIKNKVGTVQMENLESMKRKEDSYFNIRLRGFWPYAEMQNKIEFKLKQYGIEIRKVAPNNTSKTCSKCGHLNNYFNFEYRKKNKFPHFKCEKCNFKENADYNAALNISNPKLKSTKEEP

SEQ ID NO: 257 - protein, 726 aa, synthetic construct
SEVEFSHEYWMRHALTLAKRAREEREVPVGAVLVLNNRVIGEGWNRAIGLHDPTAHAEIMALRQGGLVMQNYRLIDATLYVTFEPCVMCAGAMIHSRIGRVVFGVRNSKHGAAGSLVNVLNYPGMNHRVEITGGILADECAALLCDFYRMPRQVFNAQKKAQSNINPGGSSGGSSGSETPGTSESATPKSSGGSSGGSAKNTITKALKLRIVRPYNSAEVEKIVADEKNNRERIALEKNKDKVKEACSKHLKVAAYCTTQVERNACLFCKARKLDDKFYQKLRGQFPDAVFWQEIGEIFRQLQKQAAEIYNQSLIELYYEIFIKGKGFANASSVEHYLSDVCYTRAAELFKNAAIASGLRGKVKSNFRLKELKSMKSGLPTTKSDNFPIPLVKQKGGQYTGFEISSHNDDFIIKIPFGRWQAKKEIDRYRPWEKFDFEQVRKSPKPISLLLSTQRRKRNKGWSKDEGTEAEIRKVMNGDYQTSYIEVKRGSKIGEKSAWMLNLSIDVPKIDKGVDPSIIGGIDVGVKSPLVCAINDALSRYSISDNDLFHFNKKVFARRRILLKKNRHRRAGHGAKNKLKPITILTEKSKRFRKKLIERWACEIADFFIKNKVGIVQMENLESMKRREDSYFNIRLRGFWPYAEMQNKIEFKLKQYGIEVRKVAPNNTSKTCSKCGHLNNYFNFEYRKKNKFPHFKCEKCNFKENADYNAALNISNPKLKSTKEEP

SEQ ID NO: 258 - protein, 726 aa, synthetic construct
SEVEFSHEYWMRHALTLAKRARDEREVPVGAVLVLNNRVIGEGWNRAIGLHDPTAHAEIMALRQGGLVMQNYRLTDATLYVTFEPCVMCAGAMIHGRIGRVVFGVRNSKRGAAGSLMNVLNYPGMNHCVEITEGILMDECAALLCDFYRMPRQVLNAQRKAQSSISSGGSSGGSSGSETPGASGSVTPKSSGGSSAGSTRDTITKTLKLRIVRPYNSAEVEKIVAVEKNNREKIALEKNKDKVKEACSEHLKVAAYCTTQVERSACLFCKARKLDDKFYQKLRGQFPDAVFWQEIGEIFRQLQKQAAEIYNQSLIELYYEIFIKGKGFANASSVEHYLSDVCYTRAAELFKNAAIASGLRGKVKSNFRLKELKNMKSGLPTTKSDNFPVPLVKQKGGQYTGFEISSHNDDFIIKIPFGRWQVKKEIDKYRPWEKFDFEQVRKSPKPISLLLSTQRRKRNKGWSKDEGTEAEIRKVMNGDYQISYIEVKRGSKIGEKSAWMLNLSIDVPKIDKGVDPSIIGGIDVGVKSPLICAINNAFSRYGICDNDLFRFNKKVFARRRILLKKNRHKRAGHGTKNKLKPITILTEKSGRFRKKLIERWACEIANFFIKNKVGTVQMENLESMKRKEDSYFNIRLRGFWPYAEMQNKIEFKLKQYGIKIRKVAPNNTSKTCSKCGHLNNYFSFEYRKKNKFPHFKCEKCNFKEDADYNAALNISNPKLKSTKEEP

SEQ ID NO: 259 - protein, 726 aa, synthetic construct
SEVEFSHEYWMRHALTLAKRARDEREVPVGAVLVLNNRVIGEGWNRAIGLHDPTAHAEIMALRQGGLVMQNYRLTDATLYVTFEPCVMCAGAMIHSRIGRVVFGVRNSKRGAAGSLMNVLNYPGMNHCVEITEGILVDECAALLCDFYRMPRQVLNARKKAQPSINPGGSSGGSSGSETPGTSESATPESSGGSSGGSAKNTITKTLKLRIVRPYNSAEVEKIVADEKNNREKIALEKNKDKVKEACSKHLKVAAYCTTQVERNACLFCKARRLDDKFYQKLRGQFPDAVFWQEIGEIFRQLQKQAAEIYNQSLIELYYEIFIKGKGFANASSVEHYLSDVCYTRAAELFKNAAIASGLRGKVKSNFRLKELKNMKSGLPTTKSDNFPIPLVKQKGGQYTGFEISSHNSDFIIKIPFGRWQEKEEIDKYRPWEKFDFEQVRRSPKPISLLLSTQRRKKNKGWSKDEGTEAEIRKVMNGDYQTSYIEVKRGSKIGEKSAWMLNLSIDVPKIDKGVDPSIIGGIDVGVKSPLVCAINNAFSRYSISDNDLFRFNKKMFARRRILLGKNRHKRAGHGVKNKLKPITILTEKSGRFRKKLIERWACEIADFFVKNKVGTVQMENLESMKRKEDSYFNIRLRGFWPYAEMQNKIEFKLKQYGIKVRKVAPNNTSKTCSKCGHLNNYFSFEYRKKNKFPHFKCEKCNFKEDADYNAALNISNPKLKSTKEEP

SEQ ID NO: 260 - protein, 726 aa, synthetic construct
SEVEFSHEYWMRHALTLAKRARDEREVPVGAVLVLNNRVIGEGWNRAIGLHDPTAHAEIMALRQGGLVMQNYRLTDATLYVTFEPCVMCAGAMIHSRIGRVVFGVRNSKRGAAGSLMNVLNYPGMNHCVEITEGILVDECAALLCDFYRMPRQVLNAQKKAQSSISSGGPSGGSSGSGTPGASESVTPKSSGGSSAGSTKNTITKTLKLRIVRPYNSAEVEKIVADEKNSRERIALEKNKGKVKEACSEHLKVAAYCTTQVERNACLFCKARRLDDKFYQKLRGQFPDAVFWQEIGEIFRQLQKQAAEIYNQSLIELYYEIFIKGRGFANASSVEHYLSDVCYTRAAELFKNAAIASGLRGKVKSNFRLKELKNMKSGLPTTKSDNFPIPLVKQKGGQYTGFEISSHNDDFIIKIPFGRWQAKKEIDRYRPWEKFDFEQVRKSPKPISLLLSTRRRKRNKGWSKDEGTEAEIRRVMNGDYQTSYIEVKRGSKIGEKSAWMLNLSIDVPKIDKGVDPSIIGGIDVGVKSPLVCAVNNAFSRYSISDNDLFRFNKKMFARRRILLKKNRHQRAGHGAKNKLKPITILTEKSGRFRKKLIERWACEIADFFIKNKVGTVQMENLESMKRKEDSYFNIRLRGFWPYAEMQNKIEFKLKQYGIKIRKVAPNNTSKTCSKCGHLNNYFSFEYRKKNKFPHFKCEKCNFKEDADYNAALNISNPKLKSTKEEP

SEQ ID NO: 261 - protein, 726 aa, synthetic construct
SEVEFSHEYWMRHALTLAKRARDEREVPVGAVLVLNNRVIGEGWNRAIGLHDPTAHAEIMALRQGGLVMQNYRLSDATLYVTFEPCVMCAGAMIHSRIGRVVFGVRNSKRGAAGSLMNVLNYPGMNHCVEITEGILVDECAALLCDFYRMPRQVLSAQKKAQSSISSGGSSGGSSGSETPGTSGSVTPESSGGSSGGSAKNTITKTLKLRIVRPYNSAEVEKIVADEKNNREKIALEKNKDKVKEACSEHLKVAAYCTTQVERNACLFCKARKLDDKFYQKLRGQFPDAVFWQEIGEIFRQLQKQAAEIYNQSLIELYYEIFIKGKGITNASSVEHYLSDVCYTRAAELFKNAAIASGLRGKVKSNFRLKELKNMKSSLPTTKSDNFPIPLVKQKGGQYTGFEISNHNSDFIIKIPFGRWQVKKEINKYRPWEKFDFEQVRKSPKPISLLLSTQRRKRNKGWSKDEGTEAEIRKVMNGDYQTSYIEVKRGSRIGEKSAWMLSLSIDVPKIDRGVDPSIIGGIDVGVKSPLVCAINNGLSRYSISDNDLFHFNKKMFARRRILLKKNRHRRAGHGARNKLKPITVLTEKSKRFRKKLIERWACEIANFFVKNKVGTVQMENLESMKRKEDSYFNIRLRGLWPYAEMQNKIEFKLKQYGIEVRKVAPNNTSKTCSKCGHLNNYFNFEYRKRNKFPHFKCEKCNFKENADYNAALNISNPKLKGTKEEP

SEQ ID NO: 262 - protein, 726 aa, synthetic construct
SEVEFTHEYWMRHALTLAKRARDEREVPVGAVLVLNNRVIGEGWNRAIGLHDPTAHAEIMALRQGGLVLQNYRLIDATLYVTFEPCVMCAGAMIHSRIGRVVFGVRNNKHGAAGSLVNVLNYPGMNHRVEITEGILADECAALLCDFYRMPRQVFNARKKTQSSINPGGSSGGSSGSETPGTSESATPESSGGSSGSSAKNTITKTLKLRIVRPYNSAEVEKIVADEKNNREKIALEKNKDKVKEACSKHLKVAAYCTTQVERNACLFCKARRLDDKFYQKLRGQFPDAVFWQEIGEIFRQLQKQAAEVYNQSLVELYYEILIRGKGIANASSVEHYLSDVCYTRAAELFKNAAIASGLRNKIKSNFRLKELRNMKSGLPTTKSDNFPIPLVRQKGGQYTGFEISNHDGDFIIKIPFGRWRVKKEINKHRPWEKFDFEQVRKSPKPISLLLSTQRRKRNKGWSKDEGTEAEIRKVMNGDYQTSYIEVKRGSKIGEKSAWMLNLSIDVPKIDKGVDPSIIGGIDVGVKSPLVCAINNALSRYSISDNDLFHFNKKMFARRRILLRKNRHKRAGHGAKNKLKPITIMTEKSKRFRKKLIERWACEIADFFIKNKVGTVQMENLESMKRREDSYFNIRLRGFWPYAEMQNKIEFKLKQYGIVVRKVAPNNTSKTCSKCGHLNDYFNFEYRKKNKFPHFKCEKCNFKEDADYNAALNISNPKLKSTKGEP

SEQ ID NO: 263 - protein, 726 aa, synthetic construct
SEVEFSHEYWMRHALTLAKRARDEREVPVGAVLVLNNRVIGEGWNRAIGLHDPTAHAEIMALRQGGLVMQNYRLVDATLYVTFEPCVLCAGAMVHSRIGRVVFGVRNSKRGAAGSLMNVLNYPGMNHRVEITEGILADECAALLCDFYRMPRQVFNAQKKARSNINSGGSSGGSSGSETPGTSESATPESSGGSSGGSAKNTITKTLKLRIVRPYNSAEVEKIVADEKDNRERIALEKNKGKVKEACSKHLKVAAYCTTQVGRNACLFCKARKLDDKFYQELRGQFPDAVFWQEIGEIFRQLQKQAAEIYNQSLIELYYEIFVKGKGIANTSRMEHYLSDVCYTRAAGLFKNAAIASGLRGKIKSNFRLKELKSMKSGLPTTRSDNFPIPLVKQKGGQYTGFEISNHDSDFIIKIPFGRWQVKKEIDKYRPWEKFDFEQVRKSPKPISLLLSTQRRKRNKGWSKDEGTEAEIKKVMNGDYQTSYIEVKRGSKIGEKSAWMLNLSIDVPKIDKGVDPSIIGGIDVGVKSPLVCAINNAFSRYSISDNDLFHFNKKMFARRRILLKKNRHKRAGHGAKNKLKPLTILTGKSKRFRKKLIERWACEIADFFIKNKVGTVQMENLESMKRKEDSYFNIRLRGFWPYAEMQNKIEFKLKQYGIEVRKVAPNNTSKTCSKCGHLNNYFNFEYRKKNKFPHFKCEKCNFKENADYNAALNISNPKLKSTKEEP

SEQ ID NO: 264 - protein, 726 aa, synthetic construct
SEVEFSHEYWMRHALTLAKRARDEREVPVGAILVLNNRVIGEGWNRAIGLHDPTAHAEIMALRQGGLVMQNYRLIDATLYVTFEPCVMCAGAMIHSRIGRVVFGVRNSKHGAAGSLMNVLNYPGMNHRVEITEGILADECAALLCDFYRMPRQVFNARKKAQSSINPGGPSGGSSGSETPDTSEGATPESSGGNSGGSAKNTITKTLKLRIVRPYNSAEVEKIVADEKNNREKIALEKNKDKVKEACSEHLKVAAYCTTQVERNACLFCKARKLDDKFYQKLRGQFPDAVFWQELGEIFRQLQKQTAEIYNQSLIELYYEIFIKGKGFANASSVEHYLSDVCYTRAAELFKNAAIASGLRGKVKSNFRLKELKNMRSGLPTTKSDNFPIPLVKQKGGQYTGFEISSHNDDFIIKIPFGRWQVKKEIDKYRPWEKFDFEQVRKSPKPISLLLSTQRRKRSKGWSKDEGTEAEIRRVMNGDYQTSYIEVKRGSKIGEKSAWMLNLSIGVPKIDKGVDPSIIGGIDVGVKSPLVCAINDAFSRYSISDNDLFHFNKKVFARRRILLKKNRHKRAGHGAKNKLKPISILTEKSKRFRKKLIERWACEIADFFIKNKVGTVQMENLESMKRKEDSYFNIRLRGFWPYAEMQNKIEFKLKQYGIKIRKVAPNNTSRTCSKCGHLNNYFSFEYRKKNKFPHFKCEKCNFKEDADYNAALNISNPKLKGTKEEP

SEQ ID NO: 265 - protein, 726 aa, synthetic construct
SEVEFSHEYWMRHALTLAKRARDEREVPVGAVLVLNNRVIGEGWNRAIGLHDPTAHAEIMALRQGGLVMQNYRLVDATLYVTFEPCVLCAGAMVHSRIGRVVFGVRNSKRGAAGSLMNVLNYPGMNHRVEITEGILADECAALLCDFYRMPRQVFNAQKKAQSSISSGGSSGGCSGSEMPGASEGATPKSSGGSSAGSTKNTITKTLKLRIVRPYNSAEVEKIVADEKNSREKIALERNKDKVREACSEHLKVAAYCTTQVERNACLFCKARKLDDKFYQKLRGQFPDAVFWQEIGEIFRQLQKQAAEIYNQSLIELYYEIFIKGKGFANASSVEHYLSDVCYTRAAELFKNAAIASGLRGKVKSNFRLKELKNMRSGLPTTKSDNFPIPLVKQKGGQYTGFEISSHNDDFIIKIPFGRWQVKKEIDKYRPWEKFDFEQVRKSPKPISLLLSTRRRKRNKGWSKDEGTEAEIRKVMNGDYQTSYIEVKRGSKTGEKSAWMLNLSIDVPKIDKGVDPSIIGGIDVGVKSPLVCAINNALSRYSISDNDLFRFNKKMFARRRILLKKNRHKRAGHGAKNKLKPISILTGKSERFRKKLIERWACEIADFFIKNKVGTVQMENLESMKRKEDSYFNIRLRGFWPYAEMQNKIEFKLKQYGIEIRKVAPNNTSKTCSKCGHLNNYFNFEYRKKNKFPHFKCEKCNFKENADYNAALNISNPRLKSTKEEP

SEQ ID NO: 266 - protein, 726 aa, synthetic construct
SEVEFSHEYWMRHALTLAKRARDEREVPVGAVLVLNNRVIGEGWNRAIGLHDPTAHAEIVALRQGGLVMQNYRLTEATLYVTFEPCVMCAGAMIHSRIGRVVFGVRNSKRGAAGSLMNVLNYPGMNHCVEITEGILVDECAALLCDFYRMPRQVLSAQKKARSSVSSGGSSGGSSGSETPGTSESATPGSSGGSSGGSAKNTITKTLKLRIVRPYNSAEVEKIVADEKNNREKIALEKYKDKVKEACSEHLEVAAYCTTQVERNACLFCKARKLDDKFYQKLRGQFPDAVFWQEIGEIFRQLQKQAAEIYNQSLIELYYEILIKGKGFANASSVEHYLSDVCYTRAAELFKNAAIASGLRGKVKSNFRLKELKNMKSGLPTTKSDNFPIPLVKQKGGQYTGFEISSHNDDFIIKIPFGRWQVKKEIDKYRPWEKFDFEQVRKSPKPISLLLSTQRRKRNKGWSKDEGTEAEIKKVMNGGYQISYIEVKRGSKIGEKNAWTLNLSVDVPKIDKGVDPSIIGGIDVGVKSPLVCAINNALSRYSISDNDLFHFNKKVFARRRILLKKNRHRRAGHGAKNKLKPITILTEKSKRFRKKLIERWACEIADFFIKNKVGIVQMENLESMKRREDSYFNIRLRGFWPYAEMQNKIEFKLKQYGIEIRKVAPNNTSKTCSRCGHLNNYFNFEYRRKNKFPHFKCEKCSFKENADYNAALNISNPKLKSTKEEP

SEQ ID NO: 267 - protein, 726 aa, synthetic construct
SEVEFSHEYWMRHALTLAKRARDEREVPVGAVLVLNNRVIGEGWNRAIGLHDPTAHAEIMALRQGGLVMQNYRLIDTTLYVTFEPCVMCAGAMIHSRIGRVVFGVRNNKRGAAGSLMNVLNYPGMNHRVEITEGILADECAALLCDFYRMPRRVFNAQKKAQSSINSGGSSGGGSGSDTPSTSESTTPESSGGSSGGSAKNTITKTLKLRIVRPYNSAEVEKIVADEKNNREKIALEKNKDKVKEACSKHLKVASYCTTQVERNACLFCKARKLDDKFYQKLRGQFPDAVFWQELGEIFRQLQKQAAEIYNQSLIELYYEIFIKGKGFANASSVEHYLSDVCYTRAAELFKNAAIASGLRGKVKSNFRLKELKNMKSGLPTTKSDNFPIPLVKQKGGQYTGFEISSHNDDFIIKIPFGRWQVKKEIDKYRPWEKFDFEQVRKSPKPISLLLSTQRRKRNKGWSKDEGTEAEIRKVMNGDYQTSYIEVKRGSKVGEKSAWMLSLSIDVPKIDKGVDPSTIGGIDVGVKSPLVCAINNAFCRYSISDNDLFHFNKKMFARRRILLKKSRHKRAGHGAKNKLKPISILTEKSKRFRKKLIERWACEIADFFIKNKVGTVQMENLESMKRKEDSYFNIRLRGFWPYAEMQNKIEFKLKQYGIEIRKVAPNNTSKTCSKCGHLNNYFSFEYRKKNKFPHFKCEKCNFKENADYNAALNISNPKLKSTKEEP

SEQ ID NO: 268 - protein, 726 aa, synthetic construct
SEVEFSHEYWMRHALTLAKRARDEREVPVGAVLVLNNRVIGEGWNRAIGLHDPTAHAEIMALRQGGLVMQNYRLTDATLYVTFEPCVMCAGAMIHSRIGRVVFGVRNSKRGAAGSLMNVLNYPGMNHCVEITEGILVDECAALLCDFYRMPRQVLNAQKKAQPSISSGGSSGGSSGSGTPGASESVTPKSSGGSSAGSTKNTITKTLKLRIVRPYNSAEVEKIVADEKNNREKIALEKNKDKVKEACSEHLKVAAYCTTQVERNACLFCKARKLDDKFYQKLRGQFPDAVFWQEIGEIFRQLQKQAAEIYNQSLIELYYEIFIKGRGFANAGSVEHYLSDVCYTRAAELFKNAAIASGLRGKVKSNFRLKELKNMKSGLPTTKSDNFPIPLVKQKGGQYTGFEISSHNDDFIIKIPFGRWQVKKEIDKYRPWEKFDFEQVRKSPKPISLLLSTQRRKRNKGWSKDEGTEAEIRKVMNGDYQTSYIEVKRGSKTGEKSAWMLNLSIDVPKIDKGVDPSIIGGIDVGVKFPLVCAINNAFCRYSISDNDLFHFNKKMFARRRILLKKNRYKRAGHGAKNKLKPITILTEKSKRFRKKLIERWACEIADFFIKNKVGTVQMENLESMKRREDSYFNIRLRGFWPYAEMQNKIEFKLKQYGIKIRKVAPNNTSKTCSKCGHLNNYFSFEYRKKNKFPHFKCEKCNFKEDADYNAALNISNPKLKSTKEEP

SEQ ID NO: 269 - protein, 726 aa, synthetic construct
SEVEFSHEYWMRHALTLAKRARDEREVPVGAILVLNNRVIGVGWNRAIGLHDPTAHAEIMALRQGGLVTQNYRLIDATLYVTFEPCVMCAGAMIHSRIGRVVFGVRNSKHGAAGSLVNVLNCPGMNHRVEITEGILADECAALLCDFYRMPRQVFNARKKAQSSINSGGSSGGSSGSETPGTSESPTPESSGGSPGGSAKNTITKTLQLRIVRPYNSAEVEKIVTDEKNNREKIALEKNKDKVKEACSKHLKMASYCTTQVERNACLFCKARKLDDKFYQKLRGQFPDAVFWQELGGIFRQLQKQAAEIYNQSLIELYYEIFIKGKGITNAGRVEHYLSDVCYTRAAELFKNAAIASGLRSKVRSNFRLKELKSMKSGLPTTKSDNFPIPLVKQKGGQYTGFEISSHNSDFIIKIPFGRWQVKEEIDKYRPWEKFDFEQVRKSPKPISLLLSTQRRKKNKGWSKDEGTEAEIRRVMNGDYQTSYIEVKRGSKIGEKSAWMLNLSIDVPKIDKGVDPSIIGGIDVGVKSPLVCAINNSSSRYSICDNDLFRFNKKMFARRRILLKKNRHKRAGHGAKNKLKPITILTKKSERFRKKLIERWVCEVADFFIKNKVGTVQMENLESMKRKEDSYFNIRLRGFWPYAEMQNRIELKLKQYGIEIRRVAPNNTSKTCSKCGHLNNYFNFEYRKMNKFPHFKCEKCNFKENADYNAALNISNPKLKSTKEEP

SEQ ID NO: 270 - protein, 726 aa, synthetic construct
SEVEFSHEYWMRHALTLAKRARDEREVPVGAVLVLNNRVIGEGWNRAIGLHDPTAHAEIMALRQGGLVMQNYRLANATLYVTFEPCVMCAGAMIHSRIGRVVFGVRNSKRGAAGSLMNVLNYPGMNHRVEITEGILTDECAALLCDFYRMPHQVLNAQKKAQSSINSGGSAGGSSGSETPGTSGSTTPVSSGGSSGGSAKNTITKALKLRIVRPYNSAEVEKIVADEKNNREKIALEKNKDKVKEACSKHLKVAAYCTTQVERNACLFCKARRLDDKFYQKLRGQFPDAVFWQEIGEIFRQLQKQAAEIYNQSLIELYYEIFIKGKGIANASSVEHYLSDVCYTRAAELFKNAAIASGLRNKVKSNFRLKELRSMKSGLPTTKSDNFPIPLVKQKGGQYTGFEISSHNDDFIIKIPFGRWQAKKEIDKYRPWERFDFEQVRKSPKPISLLLSTQRRKRNKGWSKDEGTEAEIRKVMNGDYQTSYIEVKRGSKTGEKSAWTLNLSIDVPKIDKGVDPSIIGGIDVGVKSPLVCAINNAFSRYSISDNDLFRFNKKMFARRRILLKKNRHKRAGHGAKNKLKPVSILTGKSERFRKKLIERWACEIADFFIKNKVGTVQMENLESMKRKEDSYFNIRLRGLWPYAEMQNKIEFKLKQYGIVVRKVAPNNTSKTCSRCGHLNNYFNFEYRKKNKFPHFKCERCNFKENADYNAALNISNPKLKSTKGEP

SEQ ID NO: 271 - protein, 726 aa, synthetic construct
SEVEFSHEYWMRHALTLARRARDEREVPVGAVLVLNNRVIGEGWNRTTGLHDPTAHAEIMALRQGGLVMQNHRLVDATLYVTFEPCVMCAGAMIHSRIGRVVFGVRNSKRGAAGSLTNVLNYPGMNHRVEITEGILADECAALLCDFYRMPRQVFNAQKKAQSSINSGGSSGGSSGSETPSTSGSATPESSGGSSGGSARNTITKTLQLRIVRPYNSAEVEKIVTDEKNNREKIALEKNKDKVKEACSKHLKMASYCTTQVERNACLFCKARKLDDKFYQKLRGQFPDAVFWQELGEILRQLQKQAAEIYNQSLIELYYEIFIKGRGFANASSVEHYLSDVCYTRAAEQFKNAAIASGLRGKVKGNFRLKELKNMKSGLPTTKSDNFPIPLVKQKGGQYTGFEISSHNDDFIIKIPFGRWQVKKEIDKYRPWEKFDFEQVRKSPKPISLLLSTQRRKRNKGWSKDEGTEAEIRKVMNGDYQTSYIEVKRGSKTGEKSAWMLNLSIDVPKIDKGVDPSIIGGIDVGVKSPLVCAINNAFSRYSISDNDLFRFNKKMFARRRILLKKNRHKRAGHGAKNKLKPISILTGKSERFRKKLIERWACEIADFFIKNKVGTVQMENLESMKRKEDSYFNIRLRGFWPYAEMQNKIEFKLKQYGIEIRKVAPNNTSKTCSKCGHLNNYFNFEYRRKNKFPHFKCEKCNFKENADYNAALNISNPKLKSTKEEP

SEQ ID NO: 272 - protein, 726 aa, synthetic construct
SEVEFSHEYWMRHALTLAKRARDEREVPVGAVLVLNNRVIGEGWNRAIGLYDPTAHAEIMALRQGGLVMQNYRLIDATLYVTFEPCVMCAGAMIHSRIGRVVFGVRNNKHGAAGSLVNVLNYPGMNHRVEITEGILADECAALLCDFYRMPRQVFNARKKAQSSINPGGSSGGSSDSETPGTSESATPESSGGSSGGSAKNTITKTLKLRIVRPYNSAEVEKIVADEKNNREKIALEKNKDKVKEACSEHLKVAAYCTTQVERNACLFCKARKLDDKFYQKLRGQFPDAVFWQEIGEIFRQLQKQAAETYNQSLIELYYEIFIKGKGFANASSVEHYLSDVCYTRAAELFKNAAIASGLRGKVKSNFRLKELKNMKSGLPTTKSDNFPIPLVKQKGGQYTGFEISSHNDDFIIKIPFGRWQVKKEIDKYRPWEKFDFEQVRKSPKPISLLLSTRRRKRNKGWSKDEGTEAEIRKVMNGDYQTSYIEVKRGSKIGEKSAWMLNLSIDVPKIDKGVDPSIIGGIDVGVKSPLVCAINNAFSRYSISDNELFHFNKKMFARRRILLKKNRHKRAGHGAKNKLKPITILTEKSKRFRKKLIERWACEIADFFIKNKVGTVQMESLESMKRKEDSYFNIRLRGFWPYAEMQNKIEFKLKQYGIKIRKVAPNNTSKTCSMCGHLNNYFSFEYRKKNKFPHFKCEKCNFKENADYNAALNISNPKLKSTKEEP

SEQ ID NO: 273 - protein, 726 aa, synthetic construct
SEVEFSHEYWMRHALTLAKRARDEREVPVGAVLVLNNRVIGEGWNRAIGLYDPTAHAEIMALRQGGLVMQNYRLTDATLYVTFEPCVMCAGAMIHSRIGRVVFGVRNSKRGAAGSLMNVLNYPGMNHCVEITEGILMDECAALLCDFYRMPRQVLNAQKKAQSSISSGGPSGGSSCSETPGASESVTPKSSGGSSTGSTKNTITKTLKLRIVRPYNSAEVEKIVADEKNSREKIALEKNKDKVKEACREHLKVAAYCTTQVERSACLFCKARKLDDRFYQKLRGQFPDAVFWQEVGEIFRQLQKQAAEIYNQSLIELYYEIFIKGRGFANAGSVEHYLSDVCYTRAAELFKNAAIASGLRGKVKSNFRLKELKNMKSGLPTTKSDNFPIPLVKQKGGQYTGFEISSHNDDFIIKIPFGRWQVKKEIDKYRPWEKFDFEQVRKSPKPISLLLSTQRRKRNKGWSKDEGTEAEIRKVMNGDYQTSYIEVKRGSKIGEKSAWMLNLSIDVPKVDKGVDPSIIGGIDVGVKSPLVCAINNAFSRYSISDNDLFHFNKKMFARRRILLKKNRHKRAGHGAKNKLKPISILTEKSKRFRKKLIERWACEIADFFIKNKVGTVQMENLESMKRKEDSYFNIRLRGFWPYAEMQNKIEFKLKQYGIEIRKVAPNNTSKTCSRCGHLNNYFNFEYRKKNKFPHFKCEKCNFKENADYNAALNISNPKLKSTKEEP

SEQ ID NO: 274 - protein, 726 aa, synthetic construct
SEVEFSHEYWMRHALTLAKRARDEREVPVGAILVLNNRVIGVGWNRAIGLHDPTAHAEIMALRQGGLVMQNYRLIDATLYVTFEPCVMCAGAMIHSRIGRVVFGVRNSKHGAAGSLVNVLNYPGMNHRVEITEGILADECAALLCDFYRMPRQVFNAQKKAQSNINPGGSSGGSSGGETPGTSESATPESSGGSSGSSAKNTITKTLKLRIVRPYNSAEVEKIVADEKNNREKIALEKNKDKVKEACSEHLKVAAYCTTQVERNACLFCKARKLDDKFYQKLRGQFPDAVFWQELGEIFRQLQKQTAEIYNQSLIELYYEIFIKGKGFANASSVEHYLSDVCYTRAAELFKNAAIASGLRGKVKSNFRLKELKNMRSGLPTTKSDNFPIPLVKQKGGQYTGFEISSHNDDFIIKIPFGRWQVKKEIDKYRPWEKFDFEQVRKSPKPISLLLSTQRRKRNKGWSKDEGTEAEIRKVMNGDYQTSYIEVKRGSKTGEKSAWMLNLSIDVPKIDKGVDPSIIGGIDVGVKSPLVCAINNAFSRYSISDNDLFRFNKKMFARRRILLKKNRHKRAGHGAKNKLKPISILTGKSERFRKKLIERWACEIADFFIKNKVGTVQMENLEGMKRKEDSYFNIRLRGFWPYAEMQNKIEFKLKQYGIKIRKVAPNNTSRTCSKCGHLNNYFNFEYRKKNKFPHFKCEKCSFKEDADYNAALNISNPKLKSTKGEP

SEQ ID NO: 275 - protein, 726 aa, synthetic construct
SEVEFSHEYWMRHALTLARRARDEREVPVGAVLVLNNRVIGEGWNRAIGLHDPTAHAEIMALRQGGLVMQNYHLVDATLYVTFEPCVLCAGAMVHSRIGRVVFGVRNNKRGAAGSLMNILNHPGMNHRVEITEGILADECAALLCDFYRMPRQVFNAQKKARSNINSGGSSGGSSGSETPGTSESPIPESSGGSSGGSAKNTITKTLKLRIVRPYNSAKVEKIVADEKNNREKIALEKNKDKVKEACSEHLKVAAYCTTQVERNACLFCKARKLDDRFYQKLRGQFPDAVFWQELGEIFRQLQRQAAEVYNQSLIELYYEIFVKGKGFANASSVEHYLSDVCYTRAAELFKNAAIASGLRGKVKSNFRLKELRSMRSGLPTTKSDNFPIPLVKQKGGQYTGFEISSHNDDFIIKIPFGRWQVKKEIDKYRPWEKFDFEQVRKSPKPISLLLSTQRRKRNKGWSKDEGTEAEIRKVMNGDYQVSYVEVKRGSKVGEKSAWMLNLSIDVPKIDKGVNPSIIGGIDVGVKSPLVCAINNALSRYSVSDNDLFRFNKKMFARRRILLKKNRHKRAGHGAKNKLKPITILTKKSERFRKKLIERWACEIADFFIKYKVGTVQMENLESMKRKEDSYFNIRLRGFWPYAEMQNKIEFKLKQYGIEIRKVAPNNTSKTCSKCGHLNNYFNFEYRKRSKFPHFKCEKCNYKEDADYNAALNISNPKLKSTKEEP

SEQ ID NO: 276 - protein, 726 aa, synthetic construct
SEVEFSHEYWMRRALTLAKRARDEREVPVGAVLVLNNRVIGVGWNRAVGLHDPTAHAEIMALRQGGLVMQNYRLIEATLYVTFEPCIMCAGAMIHSRIGRVVFGVRNSKRGAAGSLMNVLNYPGMNHRVEVTEGILADECAALLCDYYRMPRQVFNAQKKAQSSTNSGGSSDGGSGSETPGTSESATPKSSGGSSGGSAKNTITKTLKLRIVRPYNSAEVEKIVADEKSNREKIALEKNKGKVKEACSKHLEVAAYCTTQVERNACPFCRARKLDDKFYQKLRGQFPDAVFWQELGEIFRQLQKQAAEIYNQSLIELYYEIFIKGKGFANASSVEHYLSDVCYTRAAELFKNAAIASGLRGKVKSNFRLKELRNMKSGLPTTKSDNFPIPLVKQKGGQYTGFEISSHNDDFIIKIPFGRWQVKKEIDKYRPWEKFDFEQVRKSPKPISLLLSTQRRKRNKGWSKDEGTEAEIRKVMNGDYQTSYIEVKRGSKIGEKSAWMLSLSIDVPKIDKGVDPSIIGGIDVGVKSPLVCAINNAFGRYSISDNDLFRFNKKMFARRRILLKKNRHKRAGHGAKNKLKPISILTGKSERFRKKLIERWACEIADFFIKNKVGTVQMENLESMKRKEDSYFNIRLRGFWPYAEMQNKIEFKLKQYGIEIRKVAPNNTSKTCSKCGHLNNYFNFEYRKKNKFPHFKCEKCNFKENADYNAALNISNPKLKSAKEEP

SEQ ID NO: 277 - protein, 726 aa, synthetic construct
SEVEFSHEYWMRHALTLAKRARDEREVPVGAILVLNNRVIGEGWNRAIGLHDPTAHAEIMALRQGGLVMQNYRLIDATLYVTFEPCVMCAGAMIHSRIGRVVFGVRNSKRGAAGSLMNVLNYPGMNHCVAITEGILVDECAALLCDFYRMPRQVLSAQKKVQSSVSPGGSSGGSSGSDTPSTSESTTPESSGGSSGGSAKNTITKTLKLRIVRPYNSAEVEKIVADEKNNREKIALEKNKDKVKEACSEHLKVAAYCTTQVERNACLFCRARKLDDKFYQKLRGQFPDAVFWQELGEILRQLQKQAAEIYNQSLIELYYEIFIKGRGFANTSSVEHYLSDVCYTRAAELFKNAAIASGLRGKVKSNFRLKELKNMKSGLPTTKSDNFPIPLVKQKGGQYTGFEISSHNDDFIIKIPFGRWQVKKETDKYRPWEKFDFEQVRKSPKPISLLLSTQRRKRNKGWSKDEGTEAEIRKVMNGDYQTSYIEVKRGRKTGEKSAWMLNLSIDVPKIDRGVDPSIIGGIDVGVKSPLVCAINNAFSRYSISDNDLFRYNKKMFARRRILLKKNRHKRAGHGAKNKLKPITILTEKSKRFRKKLIERWACEIADFFIKNKVGTVQMENLESMKRKEDSYFNIRLRGFWPYAEMQDKIEFKLKQYGIEIRKVAPNNTSKTCSKCGHLNNYFNFEYRRKYKFPHFKCEKCNFKEDADYNAALNISNPKLKSTKEEP

SEQ ID NO: 278 - protein, 726 aa, synthetic construct
SEVEFSHEYWMRHALTLAKRARDEREVPVGAILVLNNRVIGVGWNRAIGLHDPTAHAEIMALRQGGLVMQNYRLIDATLYVTFEPCVMCAGAMIHSRIGRVVFGVRNSKHGAAGSLVNVLNYPGMNHRVEITEGILADECAALLCDYYRMPRQVFNARKKAQSSINSGGSSDGGSGSETPGTCESVTPESSGGSSGGSAKNTITKTLKLRIVRPYNSAEVEKIVADEKNNREKIALEKNEDKVKEACSKHLKMASYCTTQVERNACLFCKARKLDDKFYQKLRGQFPDAVFWQELGGIFRQLQKQAAEIYNQSLIELYYEIFIKGKGITNASRVEHYLSDVCYTRAAELFKNAAIASGLRGKVKSNFRLKELKNMKSGLPTTKSDNFPIPLVKQKGGQYTGFEISSHNDDFVIKIPFGRWQVKEEIDKYRPWEKFDFEQVRKSPKPISLLLSTQRRKRNKGWSKDEGTEAEIRKVMNGDYQTSYIEVKRGSKTGEKSAWMLNLSIDVPKIDKGVDPSIIGGIDVGVKSPLVCAINNAFSRYSISDNDLFRFNKKMFARRRILLRKNRHKRAGHGARNKLKPISILTEKSKRFRKKLIERWACEIADFFIKNKVGTVQMENLESMKRKEDSYFNIRLRGFWPYAEMQNKIEFKLKQYGIEIRKVAPNNTSKTCSKCGHLNNYFNFEYRKKNKFPHFKCEKCNFRENADYNAALNISNPKLRSTKEEP

SEQ ID NO: 279 - protein, 726 aa, synthetic construct
SEVEFSHEYWMRHALTLAKRARDEREVPVGAILVLNNRVIGEGWNRAIGLHDPTAHAEIMALRQGGLVMQNYRLTDATLYVTFEPCVMCAGAMIHSRIGRVVFGVRNSKRGAAGSLMNVLNYPGMNHCVEITEGILVDECAALLCDFYRMPRHVLNARKKAQSSISPGGSSGGSSGSETPGTSESVTPESSGGSSGGSAKNTITKTLKLRIVRPYNSAEVEKIVADEKNNREKIALEKNKDKVKEACSKHLKVAAYCTTQVERNACLFCKARKLDDKFYQKLRGQFPDAVFWQEIGEVFRQLQKQAAEIYNQSLIELYYEIFIKGKGFANASSVEHYLSDVCYTRAAELFKNAAIASGLRGKVKSNFRLKELKNMKSGLPTTKSDNFPIPLVRQKGGQYTGFEISNHDGDFIIKIPFGRWQVKKEINKHRPWEKFDFEQVRKSPKPISLLLSTQRRKRNKGWSKDEGTEAEIRKVMNGDYQTSYIEVKRGSKIGEKSAWMLNLSIDVPKIDKGVDPSIIGGIDVGVKSPLVCAINNALSRYSISDNDLFHFNKKMFARRRILLRKNRHKRAGHGAKNKLKPITIMTEKSKRFRKKLIERWACEIADFFIKNKVGTVQMENLESMKRKEDSYFNIRLRGFWPYAEMQNKIEFKLKQYGIVVRKVAPNNTSKTCSKCGHLNNHFNFEYRKMNKFPHFKCEKCNFKEDADYNAALNISNPKLKSTKGEP

SEQ ID NO: 280 - protein, 726 aa, synthetic construct
SEVEFSHEYWMRHALTLAKRARDEREVPVGAILVLNNRVIGEGWNRAIGLHDPTAHAEIMALRQGGLVMQNYRLIDATLYVTFEPCVMCAGAMIHSRIGRVVFGVRNNKHGAAGSLVNVLNYPGMNHRVEITEGILADECAALLCDFYRMPRQVFNARKKAQSSISPGGSSGGSSGGETPGTSESATPESSGGSSGGSAKNTITKTLKLRIVRPYNSAEVEKIVADEKNNREKIALEKNKDKVKEACSKHLKVAAYCTTQVERNACLFCKARKLDDKFYQKLRGQFPDAVFWQELGEILRQLQKQAAEIYNQSLIELYYEIFIKGRGFANASRVEHYLSDVCYTRAAELFKNAAIASGLRGKVKSNFRLKELKNMKSGLPTTKSDNFPIPLVKQKGGQYTGFEISSHNDDFIIKIPFGRWQVKKEIDKYRPWEKFDFEQVRKSPKPISLLLSTQRRKRNKGWSKDEGTEAEIRKVMNGDYQTSYIEVKRGGRIGEKSAWMLSLSIDVPKIDRGVDPSIIGGIDVGVKSPLVCAINNALSRYSISDNDLFHFNKKMFARRRILLKKNGHRRAGHGAKNKLKPITVLTEKSKRFRKKLIERWACEIANFFIKNKVGTVQMENLENMKRKEDSYFNIRLRGLWPYAEMQNKIEFKLKQYGIEVRKVAPNNTSKTCSKCGHLNNYFNFEYRRKYKFPHFKCEKCNFKEDADYNAALNISNPKLKSTKEEP

SEQ ID NO: 281 - protein, 726 aa, synthetic construct
SEVEFSHEYWMRHALTLAKRARDGREVPVGAVLVLNNRVIGEGWNRAIGLHDPTAHAEIMALRQGGLVTQNYRLINATLYVTFEPCAMCAGAMVHSRIGRVVFGVHNSKRGAAGSLMNVLNYPGMDHRVEITGGILADECAALLCDFYRMPRRVFNAQKKAQSSINSGGSSGGSSGSETPGTSESATPESSGGGSSGSAKNTITKTLQLRIVRPYNSAEVEKIVTDEKNNREKIALEKNKDKVKEACSKHLKMASYCTTQVERNACPFCKARKLDDKFYQKLRGQFPDAVFWQELGEILRQLQKQAAEIYNQSLIELYYEIFIKGRGFANASSVEHYLSDVCYTRAAELFKNAAIASGLRGKVKSNFRLKELKNMKSGLPTTKSDNFPIPLVKQKGGQYTGFEISSHNDDFIIKIPFGRWQVKKEIDKYRPWEKFDFEQVRKSPKPISLLLSTQGRKKNKGWSRDEGTEAEIRKVMNGDYQTSYIEVKRGSKIGEKSAWMLNLSIDVPKIDKGVDPSIIGGIDVGVKSPLVCAINNAFSRYSISDNDLFRFNKKVFARRRILLKKNRYKRAGHGTKNKLKPITILTEKSGRFRKKLIERWACEIANFFIKNKVGTVQMENLESMKRREDSYFNTRLRGFWPYAEMQSKIEFKLKQYGIKIRKVAPNNTSRTCSKCGHLNNYFNFEFRKKNKFPHFKCEKCNFKEDADYNAALNISDPKLKSTKEEP

SEQ ID NO: 282 - protein, 726 aa, synthetic construct
SEVEFSHEYWMRHALTLAKRARDEREVPVGAILVLNNRVIGVGWNRAIGLHDPTAHAEIMALRQGGLVMQNYRLTDATLYVTFEPCVMCAGAMVHSRIGRVVFGVRNNKRGAAGSLMNVLNYPGMNHRVEITEGILADECAALLCDFYRMPRQVLNAQKKARSCINPGGSSGGSSGSETPGTSESATPESSGGSSGGSAKNTITKTLKLRIVRPYNSAEVEKIVADEKDNRERIALEKNKGKVKEACSEHLKVAAYCTTQVERSACLFCKARKLDDKFYQKLRGQFPDAVFWQEIGEIFRQLQKQAAEIYNQSLIELYYEIFIKGKGFANASSVEHYLSDVCYTRAAELFKNAAIASGLRGKVKSNFRLKELKNMRSGLPTTKSDNFPIPLVKQKGGQYAGFEISSHNDDFIIKIPFGRWQVKKEIDKYRPWEKFDFEQVRKSPKPISLLLSTRRRKRNKGWSKDEGTEAEIRKVMNGDYQTSYIEVKRGSKIGEKSAWMLNLSIDVPKIDKGVDPSIIGGIDVGVKSPLVCAINNAFGRYSISDNDLFRFNKKMFARRRILLKKNRHKRAGHGAKNKLKPISILTGKSERFRKKLIERWACEIADFFIKNKVGTVQMENLESMKRKEDSYFNIRLRGFWPYAEMQNKIEFKLKQYGIEIRKVAPNNTSKTCSKCGHLNNYFNFEYRKKNKFPHFKCEKCNFKENADYNAALNISNPKLKSTKEGP

SEQ ID NO: 283 - protein, 726 aa, synthetic construct
SEDEFSHEYWMRHALTLAKRARDEREVPVGAILVLNNRVIGEGWNRTTGLHDPTAHAEIMALRQGGLVMQNHRLVDATLYVTFEPCVMCAGAMIHSRIGRVVFGVRNSKRGAAGSLTNVLNYPGMNHRVEITEGILVDECAALLCDFYRMPRQVFNPQKKAQSTINSGGSSGGSSGSETPGTSESPTPESSGGSPGGSAKNTITKTLKLRIVRPYNSAEVEKIVADEKNNREKIALEKNKDKVKEACSKHLKVAAYCTTQVERNACLFCKARKLDDKFYRKLKGQFPDAVFWQEIGEIFRQLQKQAAEIYNQSLIELYYEIFIKGKGFANASSVEHYLSDVCYTRAAELFKNAAIASGLRGKVKSNFRLKELKNMKSGLPTTKSDNFPIPLVKQKGGQYTGFEISSHNDDFIIKIPFGRWQMKKEIDKYRPWEKFDFAQVRKSPKPISLLLSTQRRKKNKGWSNDEGTEAEIRKVMNGDYQTSYIEVKRGSKIGEKSAWMLSLSIDVPKIDKGVDPSIVGGIDVGVKSPLVCAINNALGRFSISDNDLFHFNKKMFARRRILLRKNRHKRAGHGAKNKLKPITIMTEKSKRFRKKLIERWACEIADFFIKNKVGTVQMENLESMKRKEDSYFNIRLRGFWPYAEMQNKIEFKLKQYGIVVRKVAPNNTSKTCSKCGHLNNYFNFEYRKKNKFPHFKCEKCNFKEVADYNAALNISNPKLKSTKEVP

SEQ ID NO: 284 - protein, 726 aa, synthetic construct
SEEEFSHEYWMRHALTLAKRARDEREVPVGAVLVLNNRVVGEGWNRAIGLHDPTAHAEIMALRQGGLVMQNYRLSDATLYVTFEPCVMCAGAMIHSRIGRVVFGVRNSKRGAAGSLMNVLNYPGMNHCVAITEGILVDECAALLCDFYRMPRQVLSAQKKVQSSVSPGGSSGGSSGSETPGASGSVTPKSSVGSSAGSTKNTITKTLKLRIVRPYNSAEVEKIVADEKNNREKIALEENKGKVKGACSKHLKVATYCTTQVERNACLFCKARKLDDKFYQKLRGQFPDAVFWQELGEILRQLQRQAAEIYNQSLIELYYEIFIKGRGFANASSVEHYLSDVCYTRAAELFKNAAIASGLRGKVKSNFRLKELKNMKSGLPTTKSDNFPIPLVKQKGGQYTGFEISSHNDDFIIKIPFGRWQVKEEIDKYRPWEKFDFEQVRKSPKPISLLLSTQRRKRNKGWSKDEGTEAEIRKVMNGDYQTSYIEVKRGSKTGEKSAWMLNLSIDVPKIDKGVDPCIIGGIDVGVKSPLVCAINDAFSRYSISDNDLFHFNKKMFARRRILLKKNGHKRAGHGAKNKLKPITIMTEKSKRFRKKLIERWACEIADFFIKNKVGTVQMENLESMKRKEDSYFNIRLRGFWPYAEMQNKIEFKLKQYGIVVRKVAPNNTSKTCSKCGHLNNYFNFEYRKKNKFPHFKCEKCNFKENADYNAALNISNPQLKSTKGEP

SEQ ID NO: 285 - protein, 726 aa, synthetic construct
SEVEFSHEYWMRHALTLAKRARDEREVPVGAVLVLNNRVIGEGWNRAIGLHDPTAHAEIMALRQGGLVMQNYRLTDATLYVTFEPCVMCAGAMVHSRIGRVVFGVRNSKRGAAGSLMNVLDYPGMNHRVEITEGILADECAALLCDFYRMPRQVFNAQKKARPNINSGGSSGGRSGSETPGTSESATPENSGGSSGSSAKNTITKTLKLRIVRPYNSAEVEKIVADEKNNREKIALEKNKDKVKEACSKHLEVAAYCTTRVERNACLFCKARKLDDRFYQKLRGQFPDAVFWQETGEIFRQLQRQAAEIYNQSLIELYYEIFIKGKGFANASSVEHYLSDVCYTRAAELFKNAAIASGLRGKVKSNFRLKELKNMKSGLPTTKSDNFPIPLVKQKGGQYTGFEISSHNDDFIIKIPFGRWQVKKEIDKYRPWEKFDFEQVRKSPKPISLLLSTQRRKRNKGWSKDEGTEAEIRKVMNGDYQTSYIEVKRGSKIGEKSAWMLNLSIDVPKIDKGVDPSIIGGIDVGVKSPLVCAINNALSRYSISDNDLFHFNKKMFARRRILLRKNRHKRAGHGAKNKLKPITIMTEKSKRFRKKLIERWACEIADFFIKNKVGTVQMENLESMKRREDSYFNIRLRGFWPYAEMQNKIEFKLKQYGIVVRKVAPNNTSKTCSKCGHLNNYFNFEYRKKNKFPHFKCEKCNFKEDADYNAALNISNPKLKSTKGEP

SEQ ID NO: 286 - protein, 726 aa, synthetic construct
SEVEFSHEYWMRHALTLAKRARDEREVPVGAVLVLNNRVIGEGWNRAIGLHDPTAHAEIMALRQGGLVLQNYRLVDATLYVTFEPCVLCAGAMVHSRIGRVVFGARNSKRGAAGSLMNILNYPGMNHRVEITEGILADECAALLCDFYRMPRQVFNAQKKAQSSISPGGSSGGSSGSETPGTSESATPESSGSGSSGSAKNTITKTLQLRIVRPYNSAEVEKIVADEKNNREKIALEKNKDKVKEACSKHLKVASYCTTQVERNACPFCKARKLDDKFYQKLRGQFPDAVFWQELGEILRQLQKQAAEIYNQSLIELYYEIFIKGRGFANASSVEHYLSDVCYTRAAELFKNAAIASGLRGKVKSNFRLKELKNMKSGLPTTKSDNFPIPLVKQKGGRYTGFEISSHNDDFIIKIPFGRWQAKKEIDRYRPWEKFDFEQVRKSPKPISLLLSTRRRKKNKGWSKDEGTEAEIRRVMNGDYQTSYIEVKRGSKIGEKSAWMLSLSIDVPKIDKGVDPRITGGIDVGVKSPLVCAINNVLSRYSISDNDLFHFNKKMFARRRILLKKNGHKRAGHGAKNKLKPITIMTEKSKRFRKKLIERWACEIADFFIKNKVGTVQMENLESMKRKEDSYFNIRLRGFWPYAEMQNKIEFKLKQYGIEIRKVAPNNTSKTCSKCGHLNNYFNFEYRRKNKFPHFKCEKCNFKEDADYNAALNISNPKLKSTKEEP

SEQ ID NO: 287 - protein, 726 aa, synthetic construct
SEVEFSHEYWMRHALTLAKRARDEREVPVGAVLVLNNRVIGEGWNRATGQNDPTAHAEIMALRQGGLVMQNHRLIDATLYVTFEPCVMCAGAMIHSRIGRVVIGVRNSKRGAAGSLMNVLNHPGMNHRVEITEGILADECAALLCDFYRMPRQVFNAQEKAQSSINPGGSSGGSSGSKTPGTSESATPESSGGSSGGSAKNSITKTLKLRIVRPYNSAEVEKIVADEKNNREKIALEKNKDKVKEACSKHLKVAAYCTTQVERNACLFCKARKLDDKFYQKLRGQFPDAVFWQEIGEVFRQLQKQAAEIYNQSLIELYYEIFIKGKGFANASSVEHYLSDVCYTRAAELFKNAAIASGLRGKVKSNFRLKELKNMKSGLPTTKSDNFPIPLVKQKGGQYTGFEISSHNDDFIIKIPFGRWQVKKEIDKYRPWEKFDFEQVRKSPKPISLLLSTQRRKRNKGWSKDEGTEAEIRKVMNGDYQTSYIEVKRGSKIGEKSAWMLNLSIDVPKIDKGVDPSIIGGIDVGVKSPLVCAINNAFSRYSISDNDLFRFNKKMFARRRILLGKNRHKRAGHGVKNKLKPITILTEKSGRFRKKLIERWACEIADFFVKNKVGTVQMENLESMKRKEDSYFNIRLRGFWPYAEMQSKIEFKLKQYGIVVRKVAPNNTSKTCSKCGHLNNYFNFEYRKKNKFPHFKCEKCSFKENADYNAALNISNPKLKSTKREP

SEQ ID NO: 288 - protein, 726 aa, synthetic construct
SEVEFSHEYWMRHALTLAKRARDEREVPVGAVLVLNNRVIGEGWNRAIGLHDPTAHAEIMALRQGGLVMQNYRLIDATLYVTFEPCVMCAGAMIHSRIGRVVFGVRNNKHGAAGSLVNVLDYPGMNHRVEITEGILADECAALLCDFYRMPRQVFNARKKAQSSISPGGSSGGSSGSETPGTNESATPESSGGGFGGSAKNTITKTLQLRIVRPYNSAEVEKIVADEKNNREKIALEKNKDKVKEACSEHLKVAAYCTTRVDRNACLFCKARRLDDKFYQKLRGQFPDAVFWQEIGEIFRQLQKQAAEIYNQSLVELYYEILIKGKGIANASSVEHYLSDVCYTRAAELFKNAAIASGLRNKIKSNFRLKELRNMKSGLPTTKSDNFPIPLVKQKGGQYTGFGISNHNGDFIIKIPFGRWQVKKEINKHRPWEKFDFEQVRKSPKPISLLLSTQRRKRNKGWSKDEGTEAEIRKVMNGDYQTSYIEVKRGSKIGEKSAWMLNLSIDVPKIDKGVDPSIVGGIDVGVKSPLVCAVNNALGRYSISDNDLFHFNKKMFARRRILLKKNRHKRAGHGTKNKLKPITILTEKSGRFRKKLIERWACEIANFFIKNKVGTVQMENLESMKRKEDSYFNIRLRGFWPYAEMQNKIEFKLKQYGIKIRKVAPNNTSKTCSKCGHLNNYFSFEYRKKNKFPHFKCEKCNFKENADYNAALNISNPKLKSTKEEP

SEQ ID NO: 289 - protein, 726 aa, synthetic construct
SEVEFSHEYWMRHALTLAKRARDEREVPVGAVLVLNNRVIGEGWNRAIGLHDPTAHAEIMALRQGGLVMQNYRLTDATLYVTFEPCVMCAGAMIHSRIGRVVFGVRNSKRGAAGSLMNVLNYPGMNHCVEITEGILVDECAALLCDFYRMPRQVLNAQKKAQSSISSGGSSGGSSGSETPGTSESATPESSGGSSGGSAKNTITKTLKLRIVRPYNSAEVEKIVADEKDNREKIALEKNKDKVKEACSKHLKVAAYCTTQVERSACLFCKARKLDDKFYQKLRGQFPDAVFWQEIGEIFRQLQKQAAEIYNQSLIELYYEIFIKGKGFANASSVEHYLSDVCYSRAAELFKNAAVASGLRGKVKSNFRLKELKSMKSGLPTTKSDNFPIPLVRQKGGQYTGFEISSHNDDFIIKIPFGRWQVKKEIDRYRPWEKFDFEQVRKSPKPISLLLSTQRRKRNKGWSKDEGTEAEIRKVMNGDYQTSYIEVKRGSKIGEKSAWMLNLSIDVPKIDKGVDPSIIGGIDVGVKSPLVCAINNAFSRYSISDNDLFHFNKKMFARRRILLKKSKHKRAGHGAKNKLKPISILTGKSERFRKKLIERWACEIADFFIKNKVGTVQMENLESMKRKEDSYFNIRLRGFWPYAEMQNRIEFKLKQYGIEIRKVAPNNTSKTCSKCGHLNNYFNFEYRKKNKFPHFKCERCNFKENADYNAALNISNPKLKSTKEGS

SEQ ID NO: 290 - protein, 726 aa, synthetic construct
SEVEFSHEYWMRHALTLAKRARDEREVPVGAVLVLNNRVIGVGWNRAIGLHDPTAHAEIMALRQGGLVMQNYRLIDATLYVTFEPCIMCAGAMIHSRIGRVVFGVRNSKRGAAGSLMNVLNYPGMNHRVEITEGVLADECAALLCDFYRMPRQVLNAQKKAQSSINSGGSSGGGSGGETPGTSESATQESSGGSSGGSAKNTITKTLKLRIVRPYNSAEVEKIVADEKNSREKAALEENKDKVKEACSEHLKVAAYCTTQVERNACLFCKARKLDDKFYQKLRGQFPDAVFWQELGEIFRQLQKQAAEIYNQSLIELYYEIFIKGKGITNASRVEHYLSDVCYTRAAELFKNAAIASGLRSKVRSNFRLKELKNMKSGLPTTKSDNFPIPLVKQKGGQYTGFEISSHNSDFIIKIPFGRWQVKEEIDKYRPWEKFDFEQVRKSPKPISLLLSTQRRQKNKGWSKDEGTEAEIRRVMNGDYKTSYIEVKRGSKIGEKSAWMLNLSIDVPKIDKGVNPSIIGGIDVGVKSPLVCAINNAFGRYSISDNDLFHFNKKMFARRRILLKRNRHKRAGHGAKNKLKPITILTEKSKRFRRKLIERWACEIADFFIKNKVGTVQMENLESMKRKEDSYFNIRLRGFWPYAEMQDKIEFKLKQYGIEIRKVAPNNTSKTCSRCGHLNNYFNFEYRRKNKFPHFKCEKCNFKENADYNAALNISNPKLKSTKEEP

SEQ ID NO: 291 - protein, 726 aa, synthetic construct
SEVEFSHEYWMRHALTLAKRARDEREVPVGAILVLNNRVIGEGWNRAIGLHDPTAHAEIMALRQGGLVMQNYRLIDATLYVTFEPCVMCAGAMIHSRIGRVVFGVRNSKRGAAGSLMNVLNYPGMNHRVEITEGILTDECAALLCDFYRMPHQVFNARKKAQPSINPGGSSGGSSGSETPGTSESATPESSGGSSGGSAKNTITKTLQLRIVRPYNSAEVEKIVADEKNNREKIALEKNKDKVKEACSKHLKVAAYCTTQVERNACLFCKARRLDDKFYQKLRGQFPDAVFWQEIGEIFRQLQKQAAEIYNQSLVELYYEIFIKGKGIANASSVEHYLSDVCYTRAAELFKNAAIASGLRGKVKSNFRLKELKNMKSGLPTTKSDNFPIPLVKQKGGQYTGFEISSHNDDFIIKIPFGRWQVKKEIDKYRPWEKFDFEQVRKSPKPISLLLSTQRRKRNKGWSKDEGTEAEIRKVMNGDYQTSYIEVKRGSKIGEKSAWMLNLSIDVPKIDKGVDPSIIGGIDVGVKSPLVCAINNALSRYSISDNDLFHFNKKMFARRRILLKRNRHRRAGHGARNKLKPITVLAEKSKRFRKKLIERWACEIADFFVKNKVGTVQMENLESMKRKEDSYFNIRLRGFWPYAEMQNKIEFKLKQYGIKVRKVAPSNTSKTCSKCGHLNNYFNFEYRKKNKFPHFKCEKCNFKENADYNAALNISNPKLKNTKEEP

SEQ ID NO: 292 - protein, 726 aa, synthetic construct
SEVEFSHEYWMRHALTLAKRARDEREVPVGAVLVLNNRVIGEGWNRAIGLHDPTAHAEIMALRQGGLAMQNYRLVDATLYVTFEPCVLCAGAMVHSRIGRVVFGVRNSKRGAAGSLMNVLNHPGMSHRVEITGGILADECAALLCDFYRMPRQVFNAQKKAQSSINSGGSSGGGSGSDTPSTSESTTPESSGGSSGGPAKNTITKTLKLRIVRPYNSAEVEKIVADEKNNREKTALEKNKDKVKEACSEHLKVAAYCTTQVERNACQFCKARKLDDKFYQKLRGQFPDAVFWQELGGIFRQLQKQAAEIYNQSLIELYYEIFIKGKGITNASRVEHYLSDVCYTRAAELFKNAAIASGLRSKVRSNFRLKELKNMKSGLPTTKSDNFPIPLVKQKGGQYTGFEISNHNSDFIIKIPFGRWQVKKEIDKYRPWEKFDFEQVRKSPKPISLLLSTQRRKKNKGWGKDEGTEAEIRRVMNGDYQTSYIEVKRGSKIGEKSAWMLNLSIDVPKIDKGVDPSIIGGIDVGVKSPLVCAINNSSSRYSICDNDLFRFNKKMFARRRILLKKNRHKRAGHGAKNKLKPISILTEKNKRFRKKLIERWACEVADFFIKNKVGTVQMENLESMKRKEDSYFNIRLRGFWPYAEMQNRIELKLKQYGIEIRRVAPNNTSRTCSKCGHLNNYFNFEYRKKSKFPHFKCEKCNFREDADYNAALNISNPKLKSTKEEP

SEQ ID NO: 293 - protein, 726 aa, synthetic construct
SEVEFSHEYWMRHALTLAKRARDEREVPVGAILVLNNRVIGEGWNRAVGLHDPTAHAEIMALRQGGLVIQNYRLIDATLYVTFEPCVMCAGAMIHSRIGRVVFGVRNSKHGAAGSLMNVLNYPGMNHRVEITGGILADECAALLCDFYRMPHQVFNARKKAQPSISSGGSSGGSGGSETPGASESVTPKSSGGGSAGSTKNTITKTLKLRIVRPYNSAEVEKIVADEKNSRERIALEKNKDKVKEACSKHLKVAAYCTTQVERNACLFCKARKLDDRFYQKLRGQFPDAVFWQEIGEIFRQLQKQAAEVYNQSLVELYYEILIKGKGITNASRVEHYLSDVCYTRAAELFKNAAIASGLRSKVRSNFRLKELKNMKSGLPTTKSDNFPIPLVKQKGGQYTGFEISSHNSDFIIKIPFGRWQVKEEIDKYRPWEKFDFEQVRKSPKPISLLLSTQRRKKNKGWSKDEGTEAEIRRVMNGDYQTSYIEVKRGSKIGEKSAWMLNLSIDVPKIDKGVDPSIIGGIDVGVKSPLVCAVNNSFSRYSICDNDLFRFNKKMFARRRILLKKNRHKRAGHGAKNKLKPISILTEKSKRFRKKLIERWACEIADFFIKNKVGTVQIENLESMKRKEDSYFNIRLRGFWPYAEMQNKIEFKLKQYGIEIRKVAPNNTSKTCSKCGHLNSYFNFEYRKKNKFPHFKCEKCNFKENADYNAALNISNPKLKSTKEEP

SEQ ID NO: 294 - protein, 726 aa, synthetic construct
SEVEFSHEYWMRRALTLAKRARDEREVPVGAVLVLNNRVIGEGWNRAIGLHDPTAHAEIMALHQGGLVMQNYRLIDATLYVTFEPCVMCAGAMIHSRIGRVVFGARNSKRGAAGSLMNVLSYPGMNHRVEITEGILADECAALLCDFYRMPRRVFNAQKKAQSSINSGGSSGGGSGSETPSTSESTTPESSGGSSAGSTKNTITKTLKLRIVRPYNSAEVEKIVADEKNNREKIALEKNKDKVKEACSKHLKMASYCTTQVERNACPFCKARKLDDKFYQKLRGQFPDAVFWQELGGILRQLQKQAAEIYNQSLIELYYEIFIKGRGFANASSVEHYLSDVCYTRAAELFKNAAIASGLRGKVKSNFRLKELKNMKSGLPTTKSDNFPIPLVKQKGGQYTGFEVSSHNDDFIIKIPFGRWQAKKEIDKYRPWEKFDFEQVRKSPKPISLLLSTQRRKRNKGWSKDEGTEAEIRKVMNGDYQTSYIEVKRGSKTGEKSAWMLNLSIDVPKIDKGVDPSIIGGIDVGVKSPLVCAINNAFSRYCISDNDLFHFNKKMFARRRILLKKNGHKRAGHGAKNKLKPITIMTEKSKRFRKKLIERWACEIADFFIKNKVGTVQMENLESMKRKEDSYFNIRLRGFWPYAEMQNKIEFKLKQYGIVVRKVAPNNTSKTCSKCGHLNNYFNFEYRRKYKFPHFKCEKCNFKEDADYNAALNISNPKLKSTKEEP

SEQ ID NO: 295 - protein, 726 aa, synthetic construct
SEVEFSHEYWMRHALTLAKRARDEREVPVGAVLVLNNRVIGEGWNRAIGLHDPTAHAEIMALRQGGLVLQNYRLVDATLYVTFEPCVLCAGAMVHSRIGRVVFGARNSKRGAAGSLMNILNYPGMNHRVEITEGILADECAALLCDFYRMPRQVFNAQKKAQSSISSGGSSGGSSGSETPSTSESATPESSGGSSGGSAKNTITKTLKLRIVRPYNSAEVEKIVADEKNNREKIALEKNKDKVKEACSKHLKMASYCTTQVERNACLFCKARKLDDKFYQKLRGQFPDAVFWQELGGIFRQLQRQAAEIYNQSLIELYYEIFIKGKGITNASRVEHYLSDVCYTRAAELFKNAAIASGLRSKVRSNFRLKELKNMKSGLPTTKSDNFPIPLVKQKGGQYTGFEISSHNSDFIIKIPFGRWQVKEEIDKFRPWEKFDFEQVRKSPKPISLLLSTQRRKKNKGWSKDEGTEAEIRKVMNGDYQTSYIEVKRGSKTGEKSAWMLNLSFDVPKIDKGVDPRIIGGIDVGVKSPLVCAINNALSRYSISDNDLFHFNKKMFARRRILLKKNGHKRAGHGAKNKLKPITIMTEKSKRFRKKLIERWACEIADFFIKNKVGTVQMENLESMKRKEDSYFNIRLRGFWPYAEMQNKIEFKLKQYGIVVRKVAPNNTSKTCSKCGHLNNHFNFEYRKKNKFPHFKCERCNFKENADYNAALNISNPKLKSTKEEP

SEQ ID NO: 296 - protein, 726 aa, synthetic construct
SEVEFSHEYWMRHALTLAKRARDEREVPVGAVLVLNNRVIGEGWNRAIGLYDPTAHAEIMALRQGGLVMQNYRLTDATLYVTFEPCVMCAGAMIHSRIGRVVFGVRNSKRGAAGSLMNVLNYPGMNHCVEITEGILVDECAALLCDFYRMPRQVLNAQKKAQPSISSGGSSGGSSGSETPGASESVTPKSSGGGSAGSTKNTITKTLKLRIVRPYNSAEVEKIVADEKNSRERIALEKNKDKVKEACSKHLKVASYCTTQVERNACLFCKARKLDDKFYQKLRGQFPDAVFWQELGGIFRQLQKQAAEIYNQSLIELYYEIFIKGRGFANASSVEHYLSDVCYTRAAELFKNAAIASGLRGKVKSNFRLKELKNMKSGLPTTKSDNFPIPLVKQKGGQYTGFEISSHNSDFIIKIPFGRWQEKEEIDKYRPWEKFDFEQVRRSPKPISLLLSTQRRKKNKGWSKDEGTEAEIRKVMNGDYQTSYIEVKRGSKIGEKSAWMLNLSIDVPKIDKGVDPSIIGGIDVGVKSPLVCAINNAFSRYSISDNDLFHFNKKMFARRRILLRKNRHKRAGHGARNKLKPITVLTEKSERFRKKLIERWACEIANFFIKNKVGTVQMENLESMKRREDSYFNIRLRGFWPYAEMQSKIEFKLKQYGIKIRKVAPNNTSKTCSKCGHLNSYFNFEYRKKNKFPHFKCEKCNFKENADYNAALNISNPKLKSTKEVP

SEQ ID NO: 297 - protein, 726 aa, synthetic construct
SEVEFSHEYWMRHALTLAKRARDEREVPVGAVLVLNNRVIGEGWNRAIGLHDPTAHAEIMALRQGGLVMQNYRLTDATLYVTFEPCVMCAGAMIHSRIGRVVFGVRNSKRGAAGSLMNVLNYPGMSHCVEITEGILVDECAALLCDFYRMPRQVLNAQKKAQSSISSGGSSGGSGGGETPGASESVTPKSSGGSSAGSTKNTITKTLKLRIVRPYNSAEVEKIVADEKNSREKIALEKNKDKVKEACSEHLKVAAYCTTQVERSACLFCKARKLDDRFYQKLRGQFPDAVFWQEISEIFRQLQKQAAEIYNQSLIELYYEILIKGKGIANASRVEHYLSDVCYTRAAELFKNAAIASGLRSKIKSNFKLKELKNMKSGLPTTKSDNFPIPLVKQKGGQCTGFEISSHNDDFIIKIPFGRWQAKKEIDKYRPWEKFDFEQVRKSPKPISLLLSTQRRKRNKGWSKDEGTEAEIRKVMNGDYQTSYIEVKRGSKTGEKSAWMLNLSIEVPKIDKGVDPSIIGGIDVGVKSPLVCAINNAFSRYSISDNDLFRFNKKMFARRRILLRKNRHKRAGHGAKNKLKPISILTGKSERFRKKLIERWACEIADFFIKNKVGTVQMENLESMKRKEDSYFNIRLRGFWPYAEMQNKIEFKLKQYGIEIRKVAPNDTSKTCSKCGHLNNYFNFEYRKKNKFPHFKCEKCNFKEDADYNAALNISNPKLKSTKEEP

SEQ ID NO: 298 - protein, 726 aa, synthetic construct
SEVEFSHEYWMRHALTLAKRARDEREVPVGAILVLNNRVIGVGWNRAIGLHDPTAHAEIMALRQGGLVTQNYRLIDATLYVTFEPCVMCAGAMIHSRIGRVVFGVRNSKHGAAGSLVNVLNYPGMNHRVEITEGILADECAALLCDFYRMPRQVFNARKKAQSSINSGGSSGGSSGSETPGTSESATPKSSGGSSGGSAKNTITKALKLRIVRPYNSAEVEKIVADEKNNRERIALEKNKDKVKEACSKHLKVAAYCTTQVERNACLFCKARKLDDKFYQKLRGQFPDAVFWQEIGEIFRQLQKQAAEIYNQSLIELYYEIFIKGKGFANASSVEHYLSDVCYTRAAELFKNAAIASGLRGKVKSNFRLKELKNMRSGLPTTKSDNFPIPLVKQKGGQYAGFEISSHNDDFIIKIPFGRWQVKKEIDKYRPWEKFDFEQVRKSPKPISLLLSTRRRKRNKGWSKDEGTEAEIRKVMNGDYLTSYIEVKRGSKIGEKSAWMLNLSIDVPKIDKGVDPSIIGGIDVGVKSPLVCAINNAFGRYSISDNDLFHFNKKMFARRRILLKRNRHKRAGHGAKNKLKPITILTEKSKRFRKKLIERWACEIADFFIKNKVGTVQMENLESMKRKEDSYFNIRLRGFWPYAEMQNKIEFKLKQYGIEIRKVAPNNTSKTCSKCGHLNNYFNFEYRKRNKFPHFKCEKCNYKEDADYNAALNISNPKLKSTKEEP

SEQ ID NO: 299 - protein, 726 aa, synthetic construct
SEVEFSHEYWMRHALTLAKRARDEREVPVGAVLVLNNRVVGVGWNRAIGLHDPTAHAEIMALRQGGLVLQNYRLTDATLYVTFEPCVMCAGAMIHSRIGRVVFGVRNSKRGAAGSLMNVLNYPGMNHRVEITEGILADECAALLCDFYHMPRRVFNAQKKAQSSINSGGSSGGSSGSESPGTSESATPKSSGGSSGGSAKNTITKALKLRIVRPYNSAEVEKIVADEKNNRERIALEKNKDKVKEACSKHLKVASYCTTQVERNACLFCKARKLDDKFYQKLRGQFPDAVFWQELGGIFRQLQKQAAEIYNQSLIELYYEIFIKGKGITNASRVEHYLSDVCYTRAAELFKNAAIASGLRSKVRSNFRLKELKNMKSGLPTTKSDNFPIPLVKQKGGQYTGFEISSHNSDFIIKIPFGRWQEKEEIDKYRPWEKFDFEQVRRSPKPISLLLSTQRRKKNKGWSKDEGTEAEIRKVMNGDYQTSYIEVKRGSKIGEKSAWMLNLSIDVPKIDKCVDPSIIGGIDVGVKSPLVCAINNAFSRYSISDNDLFRFNKKMFARRRILLGKNRHKRAGHGVKNKLKPITILTEKSGRFRKKLIERWACEIADFFVKNKVGTVQMENLESMKRKEDSYFNIRLRGFWPYAEMQNKIEFKLKQYGIKVRKVAPNNTSKTCSKCGHLNNYFSFEYRKKNKFPHFKCEKCNFKENADYNAALNISNPKLKSTKEEP

SEQ ID NO: 300 - protein, 726 aa, synthetic construct
SEVEFSHEYWMRHALTLAKRARDEREVPVGAVLVLNNRVIGEGWNRAIGLHDPTAHAEIMALRQGGLVTQNYRLIDATLYVTFEPCVMCAGAMVHSRIGRVVFGVRNSKRGAAGSLMNVLDHPGMDHRVEITEGILADECAALLCDFYRMPRQVFNAQKKAQSSINSGGPSGGSSGSETPGASESVTPKSSGGSSAGSTKNTITKTLKLRIVRPYNSAEVEKIVADEKNNRERIALEKNKDKVREACSKHLKVASYCTTQVERNACPFCKARKLDDKFYQKLRGQFPDAVFWQELGEILRQLQKQAAEIYNQSLIELYYEIFIKGKGFANASSAEHYLSDVCYTRAAELFKNAAIASGLRGKVKSNFRLKELKNMKSGLPTTKSDNFPIPLVRQKGGKYTGFEISSHNDDFIIKIPFGRWQVKKEIDKYRPWEKFDFEQVRKSPKPISLLLSTQRRKRNKGWSKDEGTEAEIRKVMNGDYQTSYIEVKRGSKIGEKSAWMLNLSIDVPKIDKGVDPSIIGGIDVGVKSPLVCAINNAFSRYSISDNDLFHFNKKMFARRRILLKKNRHKRAGHGAKNKLKPISILTEKSKRFRKKLIERWACEIADFFIKNKVGTVQMENLESMKRKEDSYFNIRLRGFWPYAEMQNKIEFKLKQYGIEIRKVAPNNTSKTCSKCGHLNNYFNFEYRKMNKFPHFKCEKCNFKENADYNAALNISNPKLKSTKEEP

SEQ ID NO: 301 - protein, 726 aa, synthetic construct
SEVEFSHEYWMRHALTLAKRARDEREVPVGAVLVLNNRVIGGGWNRAIGLHDPTAHAEIMALRQGGLVMQNCRLVDATLYVTFEPCVMCAGAMIHSRIGRVVFGVRNSKRGAAGSLMNVLNYPGMNHRVEITEGILADECAALLCDFYCMPRQVFNAQKRAQSSINPGGSSGGSSGSETLGTSESATPESSGGSSGGSAKNTITKTLKLRIVRPYNSAEVEKIVADEKNNREKIALEKNKDKVKEACSKHLKVAAYCTTQVERNACLFCKARKLDDKFYQKLRGQFPDAVFWQEVGEIFRQLQKQAAEIYNQSLIELYYEIFIKGKGFANASSVEHYLSDVCYTRAAELFKNAAIASGLRGKVKSNFRLKELKNMRSGLPTTKSDNFPIPLVKQKGGQYTGFEISSHNDDFIIKIPFGRWQVKKEIDKYRPWEKFDFEQVRKSPKPISLLLSTQRRKRNKGWSKDEGTEAEIRKVMNGDYQTSYIEVKRGSKIGEKSAWMLNLSIDVPKIDKGVDPSIIGGIDVGVKSPLVCAINNTFSRYSISDNDLFRFNKKMFARRRILLGKNRHKRAGHGVKNKLKPITILTEKSGRFRKKLIERWACEIADFFVKNKVGTVQMENLESMKRKEDSYFNIRLRGFWPYAEMQNKIEFKLKQYGIKVRKVAPSNTSKTCSKCGHLNNYFSFEYRKKNKFPHFKCEKCNFKENADYNAALNISNPKLKSTKEEP

SEQ ID NO: 302 - protein, 726 aa, synthetic construct
SEVEFSHEYWMRHALTLAKRARDEREVPVGAVLVLNNRVIGEGWNRTTGLHDPTAHAEIMALRQGGLVMRNYRLTDATLYVTFEPCVMCAGAMIHSRIGRVVFGVRNSKRGAAGSLMNVLNYPGMNHRVEITEGILVDECAALLCDFYRMPRQVLNAQKKAQSSISPGGSSGGSSGSETPGASESVTPKSSGGSSGGSAKNTITKTLKLRIVRPYNSAEVEKIVADEKNNREKIALEKNKGKVKEACSKHLEVAAYCTTQVERNACLFCKARKLDDKFYQKLRGQFPDAVFWQELGEILRQLQKQAAEIYNQSLIELYYEIFIKGRGFANASSVEHYLSDVCYTRAAGLFKNAAIASGLRGKVKSNFRLKELKNMKSGLPTTKSDNFPIPLVKQKGGQYTGFEISNHNGDFIIKIPFGRWQVKKEIDKYRPWEKFDFAQVRKSPKPISLLLSTQRRKRNRGWSKDEGTEAEIRKVMYGDYQTSYIEVKRGSKIGEKSAWMLNLSIDVPKIDKDVDPSIIGGIDVGVKSPLVCAINNAFSRYSISDNDLFHFNKKVFARRRILLKKNRHRRAGHGAKNKLKPITILTEKSKRFRKKLIERWACEIADFFIKNKVGTVQMENLESMKRKEDSYFNIRLRGFWPYAEMQNKIEFKLKQYGIKIRKVAPNNTSRTCSECGHLNNYFSFEYRKKNKFPHFKCEKCNFKEDADYNAALNISNPKLKGTKEEL

SEQ ID NO: 303 - protein, 726 aa, synthetic construct
SEVEFSHEHWMRHALTLAKRARDEREVPVGAVLVLNNRVIGEGWNRAIGLHDPTAHAEIMALRQGGLVMQNYRLTDATLYVTFEPCVMCAGAMIHSRIGRVVFGVRNSKRGAAGSLMNVLNYPGMNHCVEITEGILMDECAALLCDFYRMPRQVLNAQKKAQSSISSGGPSGSSSCSETPGASESVTPKSSGGSSTGSTKNTITKTLKLRIVRPYNSAEVEKIVADEKNSREKIALEKNKDKVKEACSEHLKVAAYCTTQVERNACLFCKARKLDDKFYQKLGGQFPDAVFWQEIGEIFRQLQKQAAEIYNQSLVELYYEIFIKGKGFANTSSVEHYLSDVCYTRAAELFKNAAIASGLRGKVKSNFRLKELKNMKSGLPTTKSDNFPIPLVKQKGGQYTGFEVSSHNDDFIIKIPFGRWQVKKEIDKYRPWEKFDFEQVRKSPKPISLLLSTQRRKRNKGWSKDEGTEAEIRKVMNGDYQTSYIEVKRGSKIGEKSAWMLNLSIDVPKIDKGVDPSIVGGIDVGVKSPLVCAIDNALSRYSISDNDLFHFNKKMFARRRILLKKNRHKRAGHGVKNKLKPITILTEKSGRFRKKLIERWACEIADFFVKNKVGTVQMENLESMKRKEDSYFNIRLRGFWPYAEMQNKIEFKLKQYGIKVRKVAPNNTSKTCSKCGHLNNYFSFEYRKKNKFPHFKCEKCNFKENADYNAALNISNPKLKSTKEEP

SEQ ID NO: 304 - protein, 726 aa, synthetic construct
SEVEFSHEYWMRHALTLAKRARDEREVPVGAILVLNNRVIGEGWNRAIGLNDPTAHAEIMALRQGGLVMQNYRLIDATLYVTFEPCVMCAGAMIHSRIGRVVFGVRNNKHGAAGSLVNVLNYPGMGHRVEITEGILADECAALLCDFYRMPRQVLSAQKKAQSSISSGGSSGGSSGSETPGTSESATPESSGGGSSGSAKNTITKTLQLRIVRPYNSAEVEKIVADEKNNREKIALEKNKDKVKEACSKHLKVASYCTTQVERNACLFCKARKLDDKFYQKLRGQFPDAVFWQELGGIFRQLQKQAAEIYNQSLIELYYEIFIKGKGITNASRVEHYLSDVCYTRAAELFKNAAIASGLRGKVKSNFRLKELKNMKSGLPTTKSDNFPIPLVKQKGGQYTGFEISNHNSDFIIKIPFGRWQVKEEINKYRPWEKFDFEQVRKSPKPISLLLSTQRRKRNKGWSKDEGTEAEIRKVMNGDYQTSYIEVKRGSKIGEKSAWMLNLSIDVPKIDKGVDPSIIGGIDVGVKSPLVCAINNALSRYSISDNDLFHFNKKMFARRRILLRKNRHKRAGHGAKNKLKPITIMTEKSKRFRKKLIERWACEIADFFIKNKVGTVQMENLESMKRREDSYFNIRLRGFWPYAEMQNKIEFKLKQYGIVVRKVAPNNTSKTCSKCGHLNNYFNFEYRKKNKFPHFKCEKCNFKEDADYNAALNISNPELKSTKEEP

SEQ ID NO: 305 - protein, 726 aa, synthetic construct
SEVEFSHEYWMRHALTLAKRARDEREVPVGAVLVLNNRVIGEGWNRAIGLHDPTAHAEIMALRQGGLVMQNYRLIDATLYVTFEPCVMCAGAMIHSRIGRVVFGVRNNKHGAAGSLVNVLNYPGMNHRVEITEGILADECAALLCDFYRMPRQVFNARKKAQSSISPGGSSGGSRGSETPGTSESATPESSGGSSGGSAKNTITKTLKLRIVRPYNSAEVEKIVADEKNNREKIALEKNKDKVKEACSQHLKMASYCTTQVERNACLFCKARKLDDKFYQKLRGQFPDAVFWQELGGIFRQLQKQAAEIYNQSLIELYYEIFIKGKGITNASRVEHYLSDVCYTRAAELFKNAAIASGLRSKVRSNFRLKELKNMKSGLPTTKSDNFPIPLVKQKGGQYTGFEISSHNSDFVIKIPFGRWQVKEEIDKYRPWEKFDFEQVRKSPKPISLLLSTQRRKRNKGWSKDEGTEAEIRKVMNGDYQTSYIEVKRGSKIGEKSAWMLNLSIDVPKIDKGVDPSIIGGIDVGVKSPLVCAINNALSRYSISDNDLFHFNKKMFARRRILLRKNRHKRAGHGAKNKLKPITIMTERSKRFRKKLIERWACEIADFFIKNKVGTVQMENLESMKRKEDSYFNVRLRGFWPYAEMQNKIEFKLKQYGIVVRKVAPNNTSKTCSKCGHLNNYFNFEYRKKNKFPHFKCEKCNFKEDADYNAALNISNPKLKSTKGEP

SEQ ID NO: 306 - protein, 726 aa, synthetic construct
SEVEFSHEYWMRHALTLAKRARDEREVPVGAVLVLNNRVIGEGWNRTTGLHDPTAHAEIMALRQGGLVMQNHRLVDATLYVTFEPCVMCAGAMIHSRIGRVVFGVRNNKRGAAGSLMNILNYPGMNHRVEITEGILADECAALLCDFYRMPRQVFNAQKKARSNINSGGSSGGSSGSETPGTSESPTPESSGGSSGGSAKNTITKTLKLRIVRPYNSAEVEKIVADEKNNREKIALEKNKDKVKEACSEHLKVAAYCTTQVERNACLFCKARKLDDKFYQKLRGQFPGAVFWQEIGEIFRQLQKQAAEVYNQSLIELYYEIFVKGKGFANASSVEHYLSDVCYTRAAELFKNAAIASGLRGKVKSNFKLKELRSMRSGLPTTKSDNFPIPLVKQKGGQYTGFEISSHNDDFIIKIPFGRWQVKKEIDKYRPWEKFDFEQVRKSPKPISLLLSTQRRRRNKGWSKDEGTEAEIRKVMNGDYQTSYIEVKRGSKVGEKSAWMLNLSIDVPKIDKGVDPSIIGGIDVGVKSPLVCAINNAFSRYSISDNDLFRFNKKMFARRRILLKKNRHKRAGHGAKNKLKPITILTEKSGRFRKKLIERWACEIADFFIKNKVGTVQMENLESMKRKEDSYFNIRLRGFWPYAEMQSKIEFKLKQYGIEIRKVAPNNTSKTCSKCGHLNNYFNFEFRKKNKFPHFKCEKCNFKEDADYNAALNISNPKLKSTKEEP

SEQ ID NO: 307 - protein, 726 aa, synthetic construct
SEVEFSHEYWMRHALSLAKRARDEREVPVGAVLVLNNRIIGEGWNRAVGLHDPTAHAEIMALRQGGLVMQNYRLTDATLYVTFEPCVMCAGAMVHSRIGRVVFGVRNSKRGAAGSLMNVLNYPGVNHCVEITEGILVDECAALLCDFYRMPRRVLNAQKKAQSSISSGGPSGGCSGSEVPGASESVTPKSSGGSSTGSTKNTITKTLKLRIVRPYNSAEVEKIVADEKNNREKIALEKNKDKVKEACSKHLKVASYCTTQVERNACPFCKARKLDDKFYQKLRGQFPDAVFWQELGEIFRQLQKQAAEIYNQSLIELYYEIFIKGRGFANAGSVEHYLSDVCYTRAAELFKNAAIASGLRGKVKSNFRLKELKNMKSGLPTTKSDNFPIPLVKQKGGQYTGFEISSHNDDFIIKIPFGRWQVKKEIDKYRPWEKFDFEQVRKSPKPISLLLSTQRRRRNKGWGKDEGTEAEIRRVMNGDYQTSYIEVKRGSKIGEKSAWMLNLSIDVPKIDKGVDPSIIGGIDVGVKSPLVCAINNAFSRYSISDNDLFRFNKKMFARRRILLKKNRHQRAGHGAKNKLKPITILTEKSGRFRKKLIERWACEIADFFIKNKVGTVQMENLESMKRKEDSYFNIRLRGFWPYAEMQNKIEFKLKQYGIEIRKVAPNNTSKTCSKCGHLNNYFNFEYRKKNKFPHFKCEKCNFKENADYNAALNISNPKLKSTKGKP

SEQ ID NO: 308 - protein, 726 aa, synthetic construct
SEVEFSHEYWMRHALTLAKRARDEREVPVGAVLVLNNRVIGEGWNRAIGLHDPTAHAEIMALRQGGLVMQNYRLTDATLYVTFEPCVMCAGAMIHSRIGRVVFGVRNSKRGAAGSLMNVLNYPGMNHCVEITEGILVDECAALLCDFYRMPRQVLNAQKKAQSSISSGGSSGGSSGSKTPGARGSVTPKSSGGGSAGSTKDTITKTLKLRIVRPYNSAEVEKIVADEKNNREKIALEKNKDKVKEACSQHLKMASYCTTQVERNACLFCKARKLDDKFYQKLRGQFPDAVFWQELGGIFRQLQKQAAEIYNRSLIELYYEIFIKGKGFANASSVEHYLSDVCYTRAAELFKNAAIASGLRGKVKSNFRLKELKNMKSGLPTTKSDNFPIPLVKQKGGQYTGFEISSHNDDFIIKIPFGRWQVKKEIDKYRPWEKFDFEQVRKSPKPISLLLSTQRRKRNKGWSKDEGTEAEIRKVMNGDYQTSYIEVKRGSKTGEKSAWMLNLSIDVPKIDKGVDPSIIGGIDVGVKSPLVCAINNAFGRYNISDNDLFRFNKKMFARRRILLKKNGHKRAGHGARNKLKPITIMTEKSKRFRKKLIERWACEIADFFIKNRVGTVQMENLESMKRKEDSYFNIRLRGFWPYAEMQNKIEFKLKQYGIEVRKVAPNNTSKTCSKCGHLNNYFNFEYRKKNKFPHFKCEKCNFKENADYNAALNISNPKLKSTKEEP

SEQ ID NO: 309 - protein, 726 aa, synthetic construct
SEVEFSHEYWMRRALTLAKRARDEREVPVGAVLVLNNRVIGVGWNRAAGLHDPTAHAEIMALRQGGLVMQNYRLVEATLYVTFEPCIMCAGAMIHSRIGRVVFGVRNSKRGAAGSLMNVLNYPGMNHRVEITEGILVDECAALLCDFYRMPRQVLNAQKKAQSSISSGGSSGGCSGSEMPGASESVTPKSSGGSSAGSTKNTITKTLKLRIVRPYNSAEVEKIVADEKNSREKIALERNKDKVKEACSEHLKVAAYCTTQVERNACLFCKARKLDDKFYQKLRGQFPDAVFWQEIGEIFRQLQKQAAEIYNQSLIELYYEIFIKGKGFANASSVEHYLSDVCYTRAAELFKNAAIASGLRGKVKSNFRLKELKNMRSGLPTAKSDNFPIPLVKQKGGQYTGFEISSHNDDFIIKIPFGRWQVKKEIDKYRPWEKFDFEQVRKSPKPISLLLSTQRRKRNKGWSKDEGTEAEIRKVMNGDYLTSYIEVKRGSKTGEKSAWMLSLSIDVPKIDKGVDPSIIGGIDVGVKSPLVCAINNAFSRYSISDNDLFHFNKKMFARRRILLKKNRHRRAGHGAKNKLKPIAVLAEKSEGFRKKLIERWACEVADFFIKNKVGTVQMENLESMKRREDSYFNIRLRGFWPYAEMQNKIEFKLKQYGIVVRKVAPNNTSKTCSQCGHLNNYFNFEYRKKNQFPYFKCEKCNFKENADYNAALNISNPQLKSTKGEP

SEQ ID NO: 310 - protein, 726 aa, synthetic construct
SEVELSHEYWMRHALTLAKRARDEREVPVGAVLVLNNRVIGEGWNRAIGLHDPTAHAEIMALRQGGLVMQNYRLTDATLYVTFEPCVMCAGAMIHSRIGRVVFGVRNSKRGAAGSLMNVLNYPGMNHCVEITEGILVDECAALLCDFYRMPRQVLNAQKKAQSSISSGGSSGGSSGSETPGASGSVTPKSSGGSSGGSAKNTITKTLKLRIVRPYNSAEVEKIVADEKNDREKIALEKNKDKVREACSKHLKVASYCTTQVERNACPFCKARKLDDKFYQKLRGQFPDAVFWQELGEILRQLQKQAAEIYNQSLIELYYEIFIKGKGFANASSVEHYLSDVCYSRAAELFKNAAVASGLRGKVKSNFRLKELKSMKSGLPTTKSDNFPIPLVKQKGGQYTGFEISSHNDDFIIKIPFGRWQVKEEIDKYRPWEKFDFEQVRKNPKPISLLLSTQRRKRNKGWSKDEGTEAEIRKVMNGDYQTSYIEVKRGSKIGEKSAWMLNLSIDVPKIDKGVDPSIIGGIDVGVKSPLVCAINNAFSRYSISDNDLFRFNKKVFARRRILLKKNRHKRAGHGTKNKLKPITMLTEKSGRFRKKLIERWACEIANFFIKNKVGTVQMENLESMKRKEDSYFNIRLRGFWPYAEMQNKIEFKLKQYGIKIRKVAPNNTSKTCCKCGHLNHYFNFEYRKKNKFPHFKCEKCNFKEDADYNAALNISNPKLKSTKGEP

SEQ ID NO: 311 - protein, 726 aa, synthetic construct
SEVEFSHEYWMRHALTLAKRARDEREVPVGAVLVLNNRVIGEGWNRAIGLHDPTAHAEIMALRQGGLVMQNYRLIDATLYVTFEPCVMCAGAMIHSRIGRVVFGVRNNKHGAAGSLVNVLNYPGMNHRVGITEGILADECAALLCDFYRMPRQVFNARKKAQSSINPGGSSGGSSGSETLGTSESATPESSGGSSGGSAKNTITKTLKLRIVRPYNSAEVEKIVADEKNNREKIALEKNKDKVKEACSKHLKVAAYCTTQVERNACLFCKARRLDDKFYQELRGQFPDAVFWQEIGEIFRQLQKQAAEIYNQGLVELYYEILIKGKGIANASSVEHYLSDVCYTRAAELFKNAAIASGLRNKIKSNFRLKELRNMRSGLPTTKSDNFPIPLVRQKGGQYTGFEISSHNDDFIIKIPFGRWQVKKEIDKYRPWEKFDFEQVRKSPKPISLLLSTQRRKRNKGWSKDEGTEAEIRKVMNGNYQTSYIEVKRGSKTGEKSAWMLNLSIDVPKIDKGVDPSIIGGIDVGVKSPLVCAINNAFSRYSISDNDLFRFNKKMFARRRILLKKNRHKRAGHGAKNKLKPISILTEKSKRFRKKLIERWACEIADFFIKNKVGTVQMENLESMKRKEDGYFNIRLRGFWPYAEMQNKIEFKLKQYGIEIRKVAPNNTSKTCSKCGHLNNYFNFEYRKMNKFPHFKCEKCNFKEDADYNAALNISNPKLKSTKEEP

SEQ ID NO: 312 - protein, 726 aa, synthetic construct
SEVELGHEYWMRHALTLAKRARDEREVPVGAVLVLNNRVIGEGWNRAIGLHDPTAHAEIMALRQGGLVMQNYRLIDATLYVTFEPCVMCAGAMIHSRIGRVVFGVRNSKHGAAGSLVNVLNYPGMSHRVEITEGILADECAALLCDFYRMPRQVFNARKKAQSSINPGSSSGGSSGSETPGTSESTTPESSGGSSGGSAKNTITKALKLRIVRPYNSAEVEKIVADEKNNREKIALEKNKDRVKEACSEHLKVAAYCTTQVERSACLFCKARKLDDKFYQKLRSQFPDAVFWQEIGEIFRQLQKQAAEIYNQSLIELYYEIFIKGKGFANASSVEHYLSDVCYTRAAELFKNAAIASGLRGKVKSNFRLKELKNMKSGLPTTKSDNFPIPLVKQKGGQYTGFEISSRNDDFIIKIPFGRWQVKKEIDKYRPWEKFDFEQVRKSPKPISLLLSTQRRKRNKGWSKDEGTEAEIRKVMNGDYQTSYIEVKRGSKIGEKSAWMLNLSIDVPKIDKGVDPSIIGGIDVGVKSPLVCAINNALSRYSISDNDLFHFNKKMFARRRILLRKNRHKRAGHGAKNKLKPISILTERSKRFRKKLIERWACEIADFFIKNKVGTVQMENLESMKRKEDSYFNIRLRGFWPYAEMQNKIEFKLKQYGIEIRKVAPNNTSKTCSKCGHLNNYFNFEYRKKNKFPHFKCEKCNFKENADYNAALNISNPKLKSTKEEP

SEQ ID NO: 313 - protein, 726 aa, synthetic construct
SEVEFSHEYWMRHALTLAKRARDEREVPVGAVLVLNNRVIGEGWNRAVGLHDPTAHAEIMALRQGGLVMQNYRLTDATLYVTFEPCVMCAGAMIHSRIGRVVFGVRNSKRGAAGSLMNVLNYPGMNHCVEITEGILVDECAALLCDFYRMPRQVLIAQKKAQSSISSGGSSGGSSCSETPGASESVTPKSSGGSSGGSAKNTITKTLKLRIVRPYNSAEVEKIVADEKNNREKIALEKNKDKVKEACSKHLKVASYCTTQVERNACLFCKARKLDDKFYQKLRGQFPDAVFWQELGEIFRQLQKQATEIYNQSLIELYYEIFIKGKGFANASSVEHYLSDVCYTRAAELFKNAAIASGLRGKVKSNFRLKELKNMKSGLPTTKSDNFPIPLVKQKGGQYTGFEISNHNSDFIIKIPFGRWQVKKEINKYRPWEKFDFEQVRKSPKPISLLLSTQRRKRNKGWSKDEGTEAEIRKVMNGDYQTSYIEVKRGSRTGEKSAWMLSLSIDVPKIDRGVDPSIIGGIDVGVKSPLVCAINNALSRYSISDNDLFHFNKKMFARRRILLKKNGHRRAGHGARNKLKPITVLTEKSKRFRKKLIERWACEIANFFIKNKVGTVQMENLESMKRKEDSYFNIRLRGLWPYAEMQNKIEFKLKQYGIEIRKVAPNNTSKTCSKCGHLNNYFNFEYRKRNKFPHFKCEKCNFKENADYNAALNISNPKLKGTKEEP

SEQ ID NO: 314 - protein, 726 aa, synthetic construct
SEVEFSHEYWMRHALTLAKRARDEREVPVGAVLVLNNRVIGEGWNRAIGQHDPTAHAEIMALRQGGLVMQNYRLVGATLYVTFEPCVMCAGAMIHSRIGRVVFGVRNNKHGAAGSLVNVLNYPGMNHRVEITEGILADECAALLCDFYRMPRRVFSARKKAQSSINSGGSSGGNSGNKTPGTSESVTPESSGGSSGGSAKNTITKTLKLRIVRPYNSAEVEKIVADEKNNREKIALEKNKDKVKEACSKHLKVAAYCTTQVERNACQFCKARKLDDKFYQKLRGQFPDAVFWQEIGEIFRQLQKQAAEIYNQSLIELYYEIFIKGKGFANASSAEHYLSDVCYTRAAELFKNAAIASGLRGKVKSNFRLKELKNMKSGLPTTKSDNFPIPLVKQKGGKYTGFEISSHNDDFIIKIPFGRWQVKKEIDKYRPWEKFDFEQVRKSPKPISLLLSTQRRKRNKGWSKDEGTEAEIRKVMNGDYQTSYIEVKRGSKIGEKSAWMLNLSIDVPKIDKGVDPSIIGGIDVGVKSPLVCAINNAFSRYSISDNDLFHFNKKMFARRRILLKKNRHKRAGHGAKNKLKPISILTEKSKRFRKKLIERWACEIADFFIKNKVGTVQMENLESMKRKEDSYFNIRLRGFWPYAEMQNKIEFKLKQYGIEIRKVAPNNTSKTCSRCGHLNNYFNFEYRKKNKFPHFKCEKCNFKENADYNAALNISNPKLKSTKEKP

SEQ ID NO: 315 - protein, 726 aa, synthetic construct
SEVEFSHEYWMRHALTLAKRARDEREVPVGAILVLNNRVIGEGWNRAIGLHDPTAHAEIMALRQGGLVMQNYRLIDATLYVTFEPCVMCAGAMIHSRIGRVVFGVRNSKHGAAGSLVNVLNYPGMNHRVEITEGILADECAALLCDFYRMPRQVFGARRKAQSNINSGGSSGGSSGSETPGTSESPTPESSGGSSGGSAKNTITKTLKLRIVRPYNSAEVEKIVADEKNNREKIALEKNKDKVKEACSKHLMVASYCTTQVERNACPFCKARKLDDKFYQKLRGQFPDAVFWQELGEILRQLQKQAAEIYNQSLIELYYEIFIKGRGFANASSVEHYLSDVCYTRAAELFKNAAIASGLRGKVKSNFRLKELKNMKSGLPTTKSDNFPIPLVKQKGGQYTGFEISSHNDDFIIKIPFGRWQVKKEIDKYRPWEKFDFEQVRKSPKPISLLLSTQRRKRNKGWSKDEGTEAEIRKVMNGDYQTSYIEVKRGSKIGEKSAWMLNLSIDVPRIDKGVDPSIIGGIDVGVKSPLVCAINSAFSRYSISDNDLFRFNKKMFARRRILLKKNRHKRAGHGAKNKLKPISILTEKSKRFRKKLIERWACEIADFFIKNKVGTVQMENLESMKRKEDSYFNIRLRGFWPYAEMQDKIEFKLKQYGIEIRKVAPNNTSKTCSRCGHLNNYFNFEYRRKNKFPHFKCEKCNFKENADYNAALNISNPKLKSTKEEP

SEQ ID NO: 316 - protein, 726 aa, synthetic construct
SEVEFSHEYWMRHALTLAKRARDEREVPVGAVLVLNNRVIGEGWNRAIGLHDPTAHAEIMALRQGGLVMQNYRLTDATLYVTFEPCVMCAGAMIHSRIGRVVFGVRNSKRGAAGSLMNVLNYPGMNHCVEITEGILVDECAALLCDFYRMPRQVLNAQKKAQSSISPGGSSGGSSGSETPGTSESATPESSGGSSGSSAKNTITKTLKLRIVRPYNSAEVEKIVADEKDNRERIALEKNKGKVKEACSKHLKVAAYCTTQVERNACLFCKARKLDGKFYQELRGQFPDAVFWQEIGEIFRQLQKQAAEIYNQSLIELYYEILIKGKGFANACSVEHYLSDVCYTRAAELFKNAAIASGLRGKVKSNFRLKELKNMKSGLPTTKSDNFPIPLVKQKGGQYTGFEISSHNDDFIIKIPFGRWQMKKEIDRYRPWEKFDFEQVRKSPKPISLLLSTQRRKRNKGWSKDEGTEAEIRKVMNGDYQTSYIEVKRGSKMGEKSAWMLSLSIDVPKIDKGVDPSIIGGIDVGVKSPLVCAINNAFNRYSISDNNLFHFNKKMFARRRILLKKNRHKRAGHGAKNKLRPISILTEKSERFRKKLIERWACEIADFFIRNKVGTVQMENLEGMKRKEDSYFNIRLRGFWPYAEMQNKIEFKLKQYGIEVRKVAPNNTSKTCSKCGHLNNYFNFEYRKKNKFPHFKCEKCNFKENADYNAALNISNPKLKSAKEEP

SEQ ID NO: 317 - protein, 726 aa, synthetic construct
SEVEFSHEYWMRHALTLAKRARDEREVPVGAVLVLNNRVIGEGWNRAIGLHDPTAHAEIMALRQGGLVMQNYRLIDATLYVTFEPCVMCAGAMIHSRIGRVVFGVRNGKRGAAGSLMNVLNYPGMNHCVEITEGILVDECAALLCDFYRMPRQVLNAQKKAQSSISSGGSSGGSNGSETRGASESATPKSSGGSSGGSAKNTITKTLKLRIVRPYNSAEVEKIVADEKNNRERIALEKNKDKVKEACSKHLKVAAYCTTQVERNACLFCKARRLDDKFYQKLRGQFPDAVFWQEIGEIFRQLQKQAAEIYNQSLIELYYEIFIKGKGFANASSVEHYLSDVCYTRAAELFKNAAIASGLRGKVKSNFRLKELKGMKSGLPTTKSDNFPIPLVKQKGGQYTGFEISSHNDDFIIKIPFGRWQVKKEIDKYRPWEKFDFEQVRKSPKPISLLLSTQRRKRNKGWSKDEGTEAEIKRVMNGDYQTSYIEVKRGSKVGEKSAWMLNLSIDVPKIDKGVDPNIIGGIDVGVKSPLVCAINNAFSRYSISDNDLFHFNKKVFARRRILLKKNRHRRAGHGAKNKLKPITILTEKSKRFRKKLIERWACEIADFFIKNKVGTVQMENLESMKRKEDSYFNVRLRGFWPYAEMQNKIEFKLKQYGIVVRKVAPNNTSKTCSKCGHLNNYFNFEYRKKNKFPHFKCEKCNFKEDADYNAALNISNPKLKSTRGEP

SEQ ID NO: 318 - protein, 726 aa, synthetic construct
SEVEFSHEYWMRHALTLAKRARDEREVPVGAVLVLNNRVIGEGWNRAIGLHDPTAHAEIMALRQGGLVMQNYRLIDATLYVTFEPCVMCAGAMIHSRIGRVVFGVRNSKHGAAGSLVNVLNYPGMNHRVEITEGILADECAALLCDFYRMPRQVFGARRKAQSSINPGGSSGGSSGSETPGTSESPTPESPGGSSGGSAKNTITKTLKLRIVRPYNSAEVEKIVADEKNNREKIALEKNKDKVKEACSKHLKMASYCTTQVERNACLFCKARKLDDKFYQKLRGQFPDAVFWQELGGIFRQLQKQAAEIYNQSLIELYYEIFIKGKGITNASRVEHYLSDVCYTRAAELFKNAAIASGLRSKVRSNFKLKELKSMKSGLPSTKSDNFPIPLVKQKGGQYTGFEISSHDDDFIIKIPFGRWQVKKETDKYRPWEKFDFEQVRKSPKPISLLLSTQRRKRNKGWSKDEGTEAEIRKVMNGDYQTSYIEVKRGSKIGEKSAWMLNLSIDVPKIDKGVDPRIIGGIDVGVKSPLVCAINNAFSRYSISDNDLFHFNKKMFARRRILLKKNRHKRAGHGAKNKLKPITILTEKSVRFRKKLIERWACEIADFFIKNKVGTVQMENLESMKGKEDSYFNIRLRGFWPYAEMQNKIEFKLKQYGIEIRKVAPNNTSKTCSKCGHLNNYFNFEYRKKNKFPHFKCEKCHFKEDADYNAALNISNPKLRCTKEEP

SEQ ID NO: 319 - protein, 726 aa, synthetic construct
SEVEFSHEYWMRHALTLAKRARDEREVPVGAILVLNNRVIGEGWNRAIGLHDPTAHAEIMALRQGGLVMQNYRLIDATLYVTFEPCVMCAGAMVHSRIGRVVFGVRNSKRGAAGSLMNVLDYPGMGHRVEITEGILADECAALLCDFYCMPRQVFNAQKRAQSSINPGGSSGGSSGSETPGTSESATPESSGGSSGGSAKNTITKTLKLRIVRPYNSAEVEKIVADEKNNREKIALEKNKDKVKEACSEHLKVAAYCTTQVERNACLFCKARKLDDRFYQKLRGQFPDAVFWQEIGEIFRQLQKQAAEIYNQSLIELYYEIFIKGKGIANASSVEHYLSDVCYTRAAELFKNAAIASGLRNKVKSNFRLKELRSMKSGLPTTKSDNFPIPLVRQKGGQYTGFEISNHNDDFIIKIPFGRWQVKKEIDKYRPWEKFDFEQVRKSPKPISLLLSTQRRKRNKGWGKDEGTEAEIRKVMNGDYQTSYIEVKRGSKIGEKSAWMLSLSIDVPKIDKGVDPRIIGGIDVGVKSPLVCAINNALGRYSISDNDLFHFNKKMFARRRILLKKNGHKRAGHGARNKLKPITVLTEKSKRFRKKLIERWACEIAYFFIKNKVGTVQMENLESMKRKEDSYFNIRLRGFWPYAEMQNKIEFKLKQYGIEIRKVAPNNTSKTCSKCGHLNNYFNFEYRKKNKFPHFKCEKCNFKENADYNAALNISNPKLKSAKEEP

SEQ ID NO: 320 - protein, 726 aa, synthetic construct
SEVEFSHEYWMRHALTLAKRARDEREVPVGAVLVLNNRVIGGGWNRAIGLHDPTAHAEIMALRQGGLVMQNCRLVDATLYVTFEPCVMCAGAMIHSRIGRVVFGVRNSKRGAAGSLMNVLNYPGMNHRVEITEGILADECATLLCDFYRMPRQVFNARKKAQSSTNPGGSSGGSSGSEAPGTSESATPESSGSSSGGSAKNTITKTLKLRIVRPYNSAEVEKIVADEKNNREKIALEKNKDKVKEACSKHLKVASYCTTQVERNACPFCKARKLDDKFYQKLRGQFPDAVFWQELGEILRQLQKQAAEIYNQSLIELYYEIFIKGRGFANASSVEHYLSDVCYTRAAELFRNAAIASGLRGKVKSNFRLKELKNMKSGLPTTKSDNFPIPLVKQKGGQYTGFEISSHNDDFIIKIPFGRWQVKKEIDKYRPWEKFDFEQVRKSPKPISLLLSTQRRKRNKGWSKDEGTEAEIRKVMNGDYQTSYIEVKRGSKTGEKSAWMLNLSIDVPKIDKGVDPSIIGGIDVGVKSPLVCAINNAFSRYSISDNDLFRFNKKVFARRRILLGKNRHKRAGHGVKNKLKPITILTEKSKRFRKKLIERWACEIADFFIKNKVGTVQMENLESMKKREDSYFNIRLRGFWPYAEMQNKIEFKLKQYGIEIRKVAPNNTSKTCSKCGHLNNYFNFEYRKKNKFPHFKCEKCNFKENADYNAALNISNPKLKSTKEEP

SEQ ID NO: 321 - protein, 726 aa, synthetic construct
SEIEFSHEYWMRHALTLAKRARDEREVPVGAVLVLNNRVIGEGWNRAIGLHDPTAHAEIMALRQGGLVIQNYRLSDATLYVTFEPCVMCAGAMIHSRIGRVVFGARNSKRGAAGSLMNVLNYPGMNHCVEITEGILVDECAALLCDFYRMPRQVLSAQKKAQSSISSGGSSGGSSGSETPGASGSVTPKSSVGSSAGSTKNTITKTLKLRIVRPYNSAEVEKIVADEKNNREKIALEKNKDKVKEACSKHLKVASYCTTQVERNACLFCKARKLDDKFYQKLRGQFPDAVFWQELGGIFRQLQKQAAEIYNQSLIELYYEIFIKGKGIANASSVEHYLSDVCYTRAAELFKNAAIASGLRNKIKSNFRLKELRNMKSGLPTTRSDNFPIPLVRQKGGQYTGFEISNHNSDFIIKIPFGRWQVKKEIDKYRPWEKFDFAQVRKSPKPISLLLSTQRRKRNRGWSNDEGTEAEIRKVMNGDYQTSYIEVKRGSKIGEKSAWMLSLSIDVPKIDKGVDPSIVGGIDVGVKSPLVCAINNALGRFSISDNDLFHFNKKMFARRRILLRKNRHKRAGHGAKNKLKPISILTEKSRRFRKKLIERWACEIADFFIKNKVGTVQMEDLESMKRRGDSYFNIRLRGLWPYAEMQNKIEFKLKQYGIEIRKVAPNNTSKTCSKCGHLNNYFNFEYRKKNKFPHFKCEKCNFKENADYNAALNISNPKLKNTKEEP

SEQ ID NO: 322 - protein, 726 aa, synthetic construct
SEVEFSHEYWMRHALTLAKRARDEREVPVGAILVLNNRVIGEGWNRAIGLHDPTAHAEIMALRQGGLVMQNYRLIDATLYVTFEPCVMCAGAMIHSRIGRVVFGVRNNKHGAAGSLVNVLDYPGMNHRVEITEGILADECAALLCDFYRMPRQVFNARKKAQSSISLGGSSGGSSGSETPGTSESATPESSGGSSGGSAKNTITKTLTLRIVRPYNSAEVEKIVADEKNNREKIALEKNKDKVKEACSEHLKVATYCTTQVERNACLFCKARKLDDKFYQKLRGQFPDAVFWQELGEIFRQLQKQAAEIYNQSLIELYYEIFIKGKGFANASSVEHYLSDVCYTRAAELFKNAAIASGLRGKVKSNFRLKELKNMKSGLPTTKSDNFPIPLVKQKGGQYTGFEISNHNGDFIIKIPFGRWQVKKEIDKYRPWEKFDFAQVRKSPKPISLLLSTQRRKRNKGWSKDEGTEAEIKKVMNGDYQTSYIEVKRGSKTGEKSAWMLNLSIDVPKIDKGVDPSIVGGIDVGVKSPLVCAINNALGRYSISDNDLFHFNKKMFARRRILLKKNGRKRAGHGARNKLKPITVLTEKSRRFRKKLIERWACEIANFFIKNRVGTVQMENLESMKRKEDSYFNIRLRGFWPYAEMQNRIEFKLKQYGIEIRKVAPNNTSKTCSKCGHLNNYFNFEYRKKNKFPHFKCEKCNFKENADYNAALNISNPKLKSTKEEP

SEQ ID NO: 323 - protein, 726 aa, synthetic construct
SEVEFSHEYWMRHALTLAKRARDEREVPVGAVLVLNNRVIGEGWNRAIGLHDPTAHAEIMALRQGGLVMQNYRLIDATLYVTFEPCVMCAGAMVHSRIGRVVFGVRNSKRGAAGSLMNVLDYPGMDHRVKITEGILADECAALLCDFYRMPRQVFNAQKRAQSSINSGGSSGGSSGSETPGTSESATPESSGGGSSGSAKNTITKTLQLRIVRPYNSAEVEKIVTDEKNNREKIALEKNKDKVKEACSKHLKMASYCTTQVERNACLFCKARKLDDKFYQKLRGQFPDAVFWQELGGIFRQLQKQAAEIYNQSLIELYYEIFIKGKGITNASRVEHYLSDVCYTRAAELFKNAAIASGLRSKVRSNFRLKELKNMKSGLPTTKSDNFPIPLVKQKGGQYTGFEISSHNSDFIIKIPFGRWQVKEEIDKYRPWEKFDFEQVRKSPKPISLLLSTQRRKKNKGWSKDEGTEAEIRRVMNGDYQTSYIEVKRGSKVGEKSAWMLNLSIDVPKIDKGVDPSIIGGIDVGVKSPLVCAINNSSSRYSICDNDLFRFNKKMFARRRILLKKNRHKRAGHGAKNKLKPITILTKKSERFRKKLIERWVCEVADFFIKNKVGTVQMENLESMKRKEDSYFNIRLRGFWPYAEMQNRIELKLKQYGIEIRKVAPNNTSKTCSKCGHLNNYFNFEYRKKNKFPHFKCEKCNFREDADYNAALNISNPKLKSTKEEP

SEQ ID NO: 324 - protein, 726 aa, synthetic construct
SEVEFSHEYWMRHALTLAKRARDEREVPVGAVLVLNNRVIGEGWNRAIGLHDPTAHAEIMALRQGGLVMQNYRLTDATLYVTFEPCVMCAGAMIHSRIGRVVFGVRNSKRGAAGSLMNVLNYPGMNHCVEITEGILVDECAALLCDFYRMPRQVLNAQKKAQSSISSGGPSGGSSGSGTPGASESVTPKSSGGSSAGSTKNTITKTLKLRIVRPYNSAEVEKIVADEKNSRERIALEKNKGKVKEACSEHLKVAAYCTTQVERNACLFCKARRLDDKFYQKLRGQFPDAVFWQEIGEIFRQLQKQAAEVYNQSLVELYYEILIKGKGIANASSVEHYLSDVCYTRAAELFKNAAIASGLRNKIKSNFRLKELRNMKSGLPTTKSDNFPIPLVRQKGGQYTGFEISNHDGDFIIKIPFGRWRVKKEINKHRPWEKFDFEQVRKSPKPISLLLSTQRRKRNKGWSKDEGTEAEIRKVMNGDYQTSYIEVKRGSKIGEKSAWMLNLSIDVPKIDKGVDPSIIGGIDVGVKSPLVCAINNALSRYSISDNDLFHFNKKMFARRRILLRKNRHKRAGHGAKNKLKPITMMTEKSKRFRKKLIERWACEIADFFIKNKVGTVQMENLESMKRKEDSYFNIRLRGFWPYAEMQNKIEFKLKQYGIVVRKVAPNNTSKTCSKCGHLNNYFNFEYRKKNKFPHFKCEKCNFKENADYNAALNISNPKLKSTKGEP

SEQ ID NO: 325 - protein, 726 aa, synthetic construct
SEVEFSHEYWMRHALTLAKRARDEREVPVGAVLVLNNRVIGEGWNRAIGLHDPTAHAEIMALRQGGLVMQNYRLTDATLYVTFEPCVMCAGAMIHSRIGRVVFGVRNSKRGAAGSLMNVLNYPDMNHCVEITEGILVDECAALLCDFYRMPRQVLNAQKKAQSSISSGGSSGGSSGSETPGASESATPKSSGGSSAGSTKNTITKTLKLRIVRPYNSAEVEKIVADEKNNREKTALERNKDKVKEACSKHLKMAAYCTTQVERNACLFCKARKLDDKFYQKLRGQFPDAVFWQEVGEIFRQLQKQAAEIYNQSLIELYYEIFIKGKGFANASSVEHYLSDVCYTRAAELFKNAAIASGLRGKVKSNFRLKELKNMKSGLPTTKSDNFPIPLVKQKGGQYTGFEISSHNSDLIIKIPFGRWQVKEEIDKYRPWEKFDFEQVRKSPKPISLLLSTQRRKKNKGWSKDEGTEAEIRRVMNGDYQTSYIEVKRGSKIGEKSAWMLSLSIDVPKIDKGVDPSIIGGIDVGVKSPLVCAINNAFSRYSISDNDLFRFNKKVFARRRILLKKNRHKRAGHGTKNKLKPITILTEKSGRFRKKLIERWACEIANFFIKNKVGTVQMENLESMKRKEDSYFNIRLRGFWPYAEMQNKIEFKLKQYGIKIRKVAPNNTSKTCSKCGHLNHYFNFEYRKKNKFPHFKCEKCNFKEDADYNAAQNISNPKLKSTKEEP

SEQ ID NO: 326 - protein, 726 aa, synthetic construct
SEVEFSHEYWMRHALTLAKRARDEREVPVGAVLVLNNRIIGEGWNRVVGLHDPTAHAEIMALRQGGLVMQNYRLVEATLYVTFEPCIMCAGAMIHSRIGRVVFGVRNSKRGAAGSLMNVLNYPGMNHRVEIAEGILADECAALLCDFYRMPRQVFNGRKKAQSSINSGGSSGGSSGSETPGTSESPTPESSGGSPGGSAKNTITKTLKLRIVRPYNSAEVEKIVADEKNSREKIALEKNKDKVKEACSKHLKVAAYCTTQVERNACLFCKARKLDDKFYQKLRGQFPDAVFWQEIGEIFRQLQKQAAEIYNQSLIELYYEIFIKGKGFANASSVEHYLSDVCYTRAAELFKNAAIASGLRGKVKSNFRLKELKNMKSGLPTTKSDNFPIPLVKQKGGQYTGFEISSHNDDFIIRIPFGRWQVKEEIDKYRPWEKFDFEQVRKNPKPISLLLSTQRRKRNKGWSKDEGTEAEIRKVMNGDYQTSYIEVKRGSKIGEKSAWMLNLSIDVPKIDKGVDPSIIGGIDVGVKSPLVCAINNAFSRYSISDNDLFRFNKKVFARRRILLKKNRHKRAGHGTKNKLKPITILTEKSGRFRKKLIERWACEIANFFIKNRVGTVQMENLESMKRKEDSYFNIRLRGFWPYAEMQNKIEFKLKQYGIKIRKVAPNNTSKTCSKCGHLNNYFNFEYRKKNKFPHFKCEKCNFKENADYNAALNISNPQLKSTKGEP

SEQ ID NO: 327 - protein, 726 aa, synthetic construct
SEVEFSHEYWMRRALTLAKRARDEREVPVGAVLVLNNRVIGVGWNRAVGLHDPTAHAEIMALRQGGLVMQNYRLVEATLYVTFEPCIMCAGAMIHSRIGRVVFGVRNSKRGAAGSLMNVLNYPGMNHRVEITEGILADECAALLCDYYRMPRQVFNARKKAQSSINSGGSSDGGSGSETPGTSESATPESSGGSSGGSAKNTITKTLKLRIVRPYNSAEVEKIVADEKNNREKIALEKNKDKVKEACSEHLKVAAYCTTQVERSACLFCKARKLDDKFYQKLRGQFPDAVFWQEIGEIFRQLQKQAAEIYNQSLIVLYYEIFIKGKGFANASSVEHYLSDVCYTRAAELFKNAAIASGLRGKVKSNFRLKELKNMKSGLPTTKSDNFPIPLVKQKGGQYTGFEISGHNDDFIIKIPFGRWQVKKEIDKYRPWEKFDFEQVRKSPKPISLLLSTQRRKRNKGWSKDEGTEAEIRKVMNGDYQTSYIEVKRGSKTGEKSAWMLNLSIDVPKIDKGVDPSIIGGIDVGVKSPLVCAINNAFSRYSISDNDLFRFNKRMFARRRILLKKNRHRRAGHGAKNKLKPITILTEKSKRFRKKLIERWACEIADFFIRNKVGTVQMENLESMKRKEDSYFNIRLRGFWPYAEMQNKIEFKLKQYGIKIRKVAPNNTSRTCSKCGHLNNYFSFEYRKKNKFPHFKCEKCNFKEDADYNAALNISNPKLKGTKEEL

SEQ ID NO: 328 - protein, 726 aa, synthetic construct
SEVEFSHEYWMRHALTLAKRARDEREVPVGAILVLNNRVIGEGWNRAIGLHDPTAHAEIMALRQGGLVMQNYRLIDATLYVTFEPCVMCAGAMIHSRIGRVVFGVRNSKHGAAGSLVNVLNYPGMNHRVEITEGILADECAALLCNFYRMPRQVFNVRKKAQSSISSGGSSGGSSGSVTPGASGSVTPKSSGGSSAGTTKNTITKALKLRIVRPYNSAEVEKIVADEKNSREKIALEKNKDKVKEACSKHLKVAAYCTTQVERNACLFCKARRLDDKFYQKLRGQFPDAVFWQEIGEIFRQLQKQAAEIYNQSLVELYYEILIKGKGIANASSVEHYLSDVCYTRAAKLFKNAAIASGLRNKIKSNFRLKELRNMKSGLPTTKSDNFPIPLVRQKGGQYTGFEISNYNGDFVIKIPFGRWQAKREIDKYRPWEKFDFEQVRKSPKPISLLLSTQRRRRNKGWSKDEGTEAEIRKVMNGDYQTSYIEVKRGSKIGEKSAWMLNLSIDVPKIDKGVDPSIIGGIDVGVKSPLVCAINNAFSRYSISDNDLFHFNKKMFARRRILLKKNRHKRAGHGAKNKLKPISILTEKSKRFRKKLIERWACEIADFFIKNKVGTVQMENLESMKRKEDSYFNIRLRGFWPYAEMQNKIEFKLKQYGIEIRKVAPNNTSKTCSKCGHLNNYFNFEYRKKNKFPHFKCEKCNFKEDADYNAALNISNPKLKSTREEP

SEQ ID NO: 329 - protein, 726 aa, synthetic construct
SEVEFSHEYWMRHALTLAKRARDEREVPVGAILVLNNRVIGEGWNRAIGLHDPTAHAEIMALRQGGLVMQNYRLIDATLYVTFEPCVMCAGAMIHSRIGRVVFGARNSKRGAAGSLMNVLSYPGMNHRVEITEGILADECAALLCDFYRMPRQVFNARKKAQSSIDSGGSSGGGSGSETPSTSESTTPKNSGGSSGGSAKNTITKALKLRIVRPYNSAEVEKIVADEKNNREKIALEKNKDKVREACSKHLKVAAYCTTQVERNACLFCKARRLDDKFYQKLRGQFPDAVFWQEIGEIFRQLQKQAAEIYNQSLVELYYEILIKGKGIANASSVEHYLSDVCYTRAAELFKNAAIASGLRNKIKSNFRLKELRNMKSGLPTTKSDNFPIPLVKQKGGQYTGFEISSHNGDFIIKIPFGRWQVKKEIDKYRPWEKFDFEQVRKSPKPISLLLSTLRRKRNKGWSKDEGTEAEIRKVMNGDYQTSYIEVKRGSKIGEKSAWMLNLSIDVPKIDKGVDPSIIGGIDVGVKSPLVCAINNAFSRYSISDNDLFRFNKKMFARRRILLKKNRHQRAGHGAKNKLKPITILTEKSKRFRKKLIERWACEIADFFIKNKVGTVQMENLESMKRKEDSYFNIRLRGFWPYAEMQDKIEFKLKQYGIGIRKVAPNNTSRTCSKCGHLNNYFSFEYRKKNKFPHFKCEKCNFKEDADYNAALNISNPKLKSTKEEL

SEQ ID NO: 330 - protein, 726 aa, synthetic construct
SEVEFSHEYWMRHALTLAKRARDEREVPVGAVLVLNNRVIGEGWNRAIGLHDPTAHAEIMALRQGGLVMQNYRLTDATLYVTFEPCVMCAGAMIHSRIGRVVFGVRNSKRGAAGSLMNVLNYPGMNHCIEITEGILVDECAALLCDFYRMPRQVLNAQKKAQSSINSGGSSDGGSSSETPGTIESATPESSGGSSGGSAKNTITKTLKLRIVRPYNSAEVEKIVADEKNNREKIALEKNKDRVKEACSEHLKVAAYCTTQVERSACLFCKARKLDDKFYQKLRSQFPDAVFWQEIGEIFRQLQKQAAEIYNQSLIELYYEIFIKGKGFANASSVEHYLSDVCYTRAAELFKNAAIASGLRGKVKSNFRLKELKNMKSGLPTTKSDNFPIPLVKQKGGQYTGFEINSHNDDFIIKIPFGRWQVKKEIDKYRPWEKFDFEQVRKSPKPISLLLSTQRRKRNKGWSKDEGTEAEIRKVMNGDYQTSYIEVKRGSKIGEKSAWMLNLSIDVPKIDKGVDPSIIGGIDVGVKSPLVCAINNAFSRYSINDNDLFRFNKKMFARRRILLKKNRHQRAGHGAKNKLKPITILTEKSGRFRKKLIERWACEIADFFIKNKVGTVQMENLESMKRKEDSYFNIRLRGFWPYAEMQNKIEFKLKQYGIKIRKVAPNNTSKTCSKCGHLNNYFSFEYRKKNKFPHFKCEKCNFKENADYNAALNISNPKLMSTKEEP

SEQ ID NO: 331 - protein, 726 aa, synthetic construct
SEVEFSHEYWMRHALTLAKRARDEREVPVGAVLVLNNRVIGEGWNRAIGLHDPTAHAEIMALRQGGLVMQNYRLVDATLYVTFEPCVLCAGAMVHSRIGRVVFGVRNSKRGAAGSLMNVLNYPGMNHRVEITEGILADECAALLCDFYRMPRQVFNARKKARSNINSSGSSGGSSGSETPGTSESATPESFGGSSGGSAKNTITKTLKLRIVRPYNSAEVEKIVADEKNNREKIALEKNKDKVKEACSKHLKVAAYCTTQVERNACLFCKARKLDDKFYQKLRGQFPDAVFWQEIGEIFRQLQKQAAEIYNQGLIELYYEIFIKGKGFANASSVEHYLSDVCYTRAAELFKNAAIASGLRGKVKSNFRLKELKNMKSGLPTTKSDNFPIPLVKQKGGQYTGFEISSHNDDFIIKIPFGRWQVKKEIDKYRPWEKFDFEQVRKSPKPISLLLSTQRRKRNKGWSKDEGTEAEIRKVMNGDYQTSYIEVKRGSKTGEKSAWMLNLSIDVPKIDKGVDPSIIGGIDVGVKSPLVCAINNALSRYSISDNDLFRFNKKMFARRRVLLKKNRHKRAGHGAKNKLKPISILTEKSKRFRKKLIERWACEIADFFIKNKVGTVQIENLESMKRKEDSYFNIRLRGFWPYAEMQNKIEFKLKQYGIEIRKVAPNNTSKTCSKCGHLNNYFNFEYRKKNKFPHFKCEKCNFKENADYNAALNISNPKLKSTKKEP

SEQ ID NO: 332 - protein, 726 aa, synthetic construct
SEVEFSHEYWMRHALSLAKRARDEREVPVGAVLVLNNRIIGEGWNRAIGLHDPTAHAEIMALRQGGLVMQNYRLIDATLYVTFEPCVMCAGAMIHSRIGRVVFGVRNNKHGAAGSLVNVLNYPGMNHRVEITEGILADECAALLCDFYRMPRQVFNARKKAQSSISPGGSSGGSSGSETPGTSESAAPKSSGGSSGGSAKNTITKTLKLRIVRPYNSAEVEKIVADEKNNREKIALEKNKDKVKEACSEHLKVAAYCTTQVERSACLFCKARKLDDKFYQKLRGQFPDAVFWQEIGEIFRQLQKQAAEIYNQSLIELYYEIFIKGKGFANASSVEHYLSNVCYTRAAELFKNAAIASGLRGKVKSNFRLKELKNMKSGLPTTKSDNFPIPLVKQKGGQYTGFEISSHNDDLIVKIPFGRWQVKKEIDRYRPWEKFDFEQVRKSPKPISLLLSTQRRKRNKGWSKDEGTEAEIRKVMNGGYQTSYIEVKRGSKIGEKSAWMLSLSIDMPKIDKGVDPSIIGGIDVGVKSPLVCAINNTLSRYSISDNDLFHFNKKMFARRRILLRKNRHKRAGHGAKNKLKPITIMTEKSKRFRKKLIERWACEIADFFIKNKVGTVQMENLESMKRKEDSYFNIRLRGFWPYAEMQNKIEFKLKQYGIVVRKVAPNNTSKTCSKCGHLNNYFNFEYRKKNKFPHFKCEKCNFKEDADYNAALNISNPKLKSTKGEP

SEQ ID NO: 333 - protein, 726 aa, synthetic construct
SEVEFSHEYWMRHALTLAKRARDEREVPVGAVLVLNNRVIGVGWNRAIGLHDPTAHAEIMALRQGGLVVQNYRLTDATLYVTFEPCVMCAGAMVHSRIGRVVFGVRNSKRGAAGSLMNVLNYPGMSHRVEITEGILVDECAALLCDFYRMPRQVLNAQKKAQSSISSGGSSGGSGGGETPGASESVTPKNSGGSSAGSTKNTITKTLKLRIVRPYNSAEVEKIVADEKNNREKVALEKNKDKVKEACSEHLKVAAYCTTQVERNACLFCKARKLDDKFYQKLRGQFPDAVFWQELGGIFRQLQKQAAEIYNQSLIELYYEIFIKGKGFANASSVEHYLSDVCYTRAAELFKNAAIASGLRGKVKSNFRLKELKNMKSGLPTTKSDNFPIPLVKQKGGQYTGFEISNRNSDFIIKIPFGRWQVKKEIDKYRPWEKFDFEQVRKSPKPISLLLSTRRRKRNKGWSKDEGTEAEIRKVMNGDYQTSYIEVKRGSKIGEKSAWMLNLSIDVPRIDKGVDPSIIGGIDVGVKSPLVCAINNAFGRYSISDNDLFRFNKKMFARRRILLKKNRHKRAGHGAKNKLKPISILTGKSERFRKKLIERWACEIADFFIKNKVGTVQMENLESMKRREDSYFNIRLRGFWPYAEMQNKIEFKLKQYGIEIRKVAPNNTSKTCSKCGHLNNYFNFEYRKKNKFPHFKCEKCNFKENADYNAALNISNPKLKSTKEEP

SEQ ID NO: 334 - protein, 726 aa, synthetic construct
SEVEFSHEYWMRHALTLAKRARDEREVPVGAILVLNNRVIGEGWNRAIGLNDPTAHAEIMALRQGGLVMQNYRLIDATLYVTFEPCVMCAGAMIHSRIGRVVFGVRNNKHGAAGSLVNVLNYPGMNHRVEITEGILADECAALLCDFYRMPRQVFNARKKAQSSINPGGSSGGSGGSETPGTSESATPESSGGSSGSSAKDTITKTLKLRIVRPYNSAEVEKIVADEKNNREKIALEKNKDKVKEACSKHLKVAAYCTTQVERNACLFCKARRLDDKFYQKLRGQFPDAVFWQEIGEIFRQLQKQAAEIYNQSLVELYYEILIKGKGITNASRVEHYLSDVCYTRAAELFKNAAIASGLRSKVRSNFRLKELKNMKSGLPTTKSDNFPIPLVKQKGGQYTGFEISSHNSDFIIKIPFGRWQVKEEIDKYRPWEKFDFEQVRKSPKPISLLLSTQRRKKNKGWSKDEGTEAEIRRVMNGDYQTSYIEVKRGSKIGEKSAWVLNLSIDVPKIDKGVDPSIIGGIDVGVKSPLVCAINNSSSRYSICDNDLFHFNKKMFARRRILLKKNRHKRAGHGAKNKLKPITILTEKSKRFRKKLIERWASEIADFFIKNKVGTVQMENLESMKRKEDSYFNIRLRGFWPYAEMQNKIEFKLKQYGVEIRKVAPNNTSKTCSKCGHLNNYFNFEYRKKNKFPHFKCEKCNFKENADYNAALNISNPKLKSTKEEH

SEQ ID NO: 335 - protein, 726 aa, synthetic construct
SEVEFSHEYWMRHALTLAKRARDEREVPVGAILVLNNRVIGEGWNRAIGLHDPTAHAEIMALRQGGLVMQNYRLIDATLYVTFEPCVMCAGAMIHSRIGRVVFGVRNNKHGAAGSLVNVLDYPGMNHRVEITEGILADECAALLCDFYRMPRQVFNARKKAQSSINSGGSSGGSSGSETPGTSESATPKSSGGSSAGSTKNTVTKTLKLRIVRPYNSTEVEKIVADEKNSREKIALERNKDKVKEACSEHLKVAAYCTTQVERNACLFCKARKLDDRFYQKLRGKFPDAVFWQETGEIFRQLQRQAAEIYNQSLIELYYEIFIKGKGFANASSVEHYLSDVCYTRAAELFKNAAIASGLRGKVKSNFRLKELKNMKSGLPTTKSDNFPIPLVKQKGGQYTGFEISSHNDDFIIKIPFGKWQVKKEIDKYRPWEKFDFEQVRKSPKPISLLLSTQRRKRNKGWSKDEGTEAEIRKVMNGDYQTSYIEVKRGSKIGEKSAWMLNLSIDVPKIDKGVDPSIIGGIDVGVKSPLVCAINNAFSRYSISDNDLYRFNKKMFARRRILLKKSRHKRAGHGAKNKLKPITILTEKSGRFRKKLIERWACEIADFFIKNKVGTVQMENLESMKRKEDSYFNIRLRGFWPYAEMQNKIEFKLKQYGIEIRKVAPNNTSKTCSKCGHLNSYFNFEYRKKNKFPHFKCEKCNFKENADYNAALNISNPKLKSTKEEP

SEQ ID NO: 336 - protein, 726 aa, synthetic construct
SEVEFSHEYWMRHALTLAKRARDEREVPVGAVLVLNNRVIGEGWNRAIGLHDPTAHAEIMALRQGGLVMQNYRLTDATLYVTFEPCVMCAGAMIHSRIGRVVFGVRNSKRGAAGSLMNILNYPGMNHRVEITEGILVDECAALLCDFYRMPCQVLNAQKKAQSSISSGGSSGGSSGGDTLGASESVTPKSSVGSSASSTKNTITKTLKLRIVRPYNSAEVEKIVADEKNNREKIALEKNKDKVKEACSKHLKVAAYCTTLVERNACLFCKARKLDDKFYQKLRGQFPDAVFWQEIGEIFRQLQKQAAEIYNQCLIELYYEIFIKGKGFANASSVEHYLSDVCYTRAAELFKNAAIASGLRGKVKSNFRLKELKNMKSGLPTTKSDNFPIPLVKQKGGQYTGFEISSHNDDFIIKIPFGRWQVKKEIDKFRPWEKFDFEQVRKSPKPISLLLSTQRRKRNKGWGKDEGTEAEIRKVMNGDYQTSYIEVKRGSKTGEKSAWMLNLSIDVPKIDKGVDPSIIGGIDVGVKSPLVCAINNAFGRYSISDNDLFRFNKKMFARRRILLKKNRHKRAGHGTKNKLKPITILTEKSGRFRKKLIERWACEIANFFIKNKVGTVQMENLESMKRKEDSYFNIRLRGFWPYAEMQNKIEFKLRQYGIKIRKVAPNSTSKTCSKCGHLNNYFSFEYRKKNKFPHFKCEKCNFKEDADYNAALNISNPKLKSTKEEP

SEQ ID NO: 337 - protein, 726 aa, synthetic construct
SEVEFSHEYWMRHALTLAKRARDEREVPVGAVLVLNNRVIGEGWNRAIGLHDPTAHAEIMALRQGGLVMQNYRLVNATLYVTFEPCVMCAGAMIHSRIGRVVFGVRNSKRGAAGSLMNVLNYPGMNHRVEITEGILTDECAALLCDFYRMPHQVLNAQKKAQSSINSGGSAGGSSGSETPGTSGSATPEGSGGSSGGFAKNTITKTLKLRIVRPYNSAEVEKIVADEKNNREKIALEKNKDKVKEACSKHLKVASYCTTQVERNACPFCRARKLDDKFYQKLRGQFPDAVFWQELGEILRQLQKQAAEIYNQSLIELYYEIFIKGKGFANASSVEHYLSDVCYARAAELFKNAAIASGLRGKVKSNFRLKELKNMRSGLPTTKSDNFPIPLVKQKGGQYTGFEISSHNDDFIIKIPFGRWQVKKEIDKYRPWEKFDFEQVRKSPKPISLLLSTQRRKRNKGWSKDEGTEAEIRKVMNGDYQTSYIEVKRGSKTGEKSTWMLNLSIDVPKIDKGVDPSIIGGIDVGVKSPLVCAINNAFSRYSISDNDLFRFNKKMFARRRILLKKNRHKRAGHGAKNKLKPISILTGKSERFRKKLIERWACEIADFFIKNKVGTVQMENLESMKRKEDSYFNIRLRGFWPYAEMQNKIEFKLKQYGIEIRKVAPNNTSKTCSKCGHLNNYFNFEYRKKNKFPHFKCEKCNFKENADYNAALNISNPKLKSTKEEP

SEQ ID NO: 338 - protein, 726 aa, synthetic construct
SEVEFSHEYWMRHALTLAKRARDEREVPVGAVLVLNNRVIGEGWNRAIGLHDPTAHAEIMALRQGGLVMQNYRLIDATLYVTFEPCVMCAGAMIHSRIGRVVFGVRNSKRGAAGSLMNVLNYPGMNHCVEITEGILVDECAALLCDFYRMPRQVLNAQKKAQSSIRPGGSSGGSSGSETPGASESVTPKSSGGSSGSSAKNTITKTLKLRIVRPYNSAEVEKIVADEKNNREKIALEKNKGKVKEACSKHLEVAAYCTTQVERNACLFCKARKLDDKFYQKLRGQFPDAVFWQELGEIFRQLQKQAAEIYNQSLIELYYEIFIKGKGLANASSVEHYLSDVCYTRAAELFKNAAIASGLRGKVKSNFRLKELKNMKSGLPTTKSDNFPIPLVKQKGGQYTGFEISSHNSDFIIKIPFGRWQVKEEIDKYRPWEKFDFEQVRKSPKPISLLLSTQRRKKNKGWSKDEGTEAEIRRVMNGDYQTSYIEVKRGSKIGEKSAWMLNLSIDVPKIDKGVDPSIIGGIDVGVRSPLVCAINNAFSRYSISDNDLFHYNKKMFARRRILLKKNRHKRTGHGAKNKLKPISILTEKSKRFRKKLIERWACEIADFFIKNKVGTVQIENLEGMKRKEDSYFNIRLRGFWPYAEMQNKIEFKLKQYGIEIRKVAPNNTSKTCSKCGHLNSYFNFEYRKKNKFPHFKCKKCNFKENADYNAALNISNPKLKSTKEEP

SEQ ID NO: 339 - protein, 726 aa, synthetic construct
SEVEFSHEYWMRHALTLAKRARDEREVPVGAVLVLNNRVIGEGWNRAIGLHDPTAHAEVMALRQGGLVMQNYRLIDATLYVTFEPCVMCAGAMIHSRIGRVVFGARNSKRGAAGSLMNVLSYPGMNHRVEITEGILADECAALLCDFYRMPRRVFNAQKKAQSSINSCGSSGGGSGSETPSTSESTTPESSGGSSGGPAKNTITKTLKLRIVRPYNSAEVEKIVADEKNNREKTALEKNRDKVKEACSEHLKVAAYCTTQVERNACLFCKARKLDDRFYQKLRGQFPDAVFWQETGEIFRQLQRQAAEIYNQSLIELYYEIFIKGKGFANASSVEHYLSDVCYTRAAELFKNAAIASGLRGKVKSNFRLKELRSMRSGLPTTKSDNFPIPLVKQKGGQYTGFEISSHNDDFIIKIPFGRWQVKKEIDKYRPWEKFDFEQVRKNPKPISLLLSTQRRKRNKGWSKDEGTEAEIRKVMNGDYQTSYIEVKRGSKIGEKSAWVLNLSIDVPKIDKGVDPSIIGGIDVGVKSPLVCAINNAFSRYSISDNDLFRFNKKVFARRRILLKKNRHKRAGHGTKNKLKPITILTEKSGRFRKKLIERWACEIANFFIKNKVGTVQMENLEGMKRKEDSYFNIRLRGFWPYAEMQNKIEFKLKQYGIKIRKVAPNNTSKTCSKCGHLNNYFSFEYRKKNKFPHFKCEKCNFKEDADYNAALNISNPKLKSTKEEP

SEQ ID NO: 340 - protein, 726 aa, synthetic construct
SEVEFSHEYWMRHALTLAKRARDEREVPVGAVLVLNNRVIGEGWNRAIGLHDPTAHAEIMALRQGGLVMQNYRLTDATLYVTFEPCIMCAGAMIHSRIGRVVFGVRNSKRGAAGSLMNVLNYPGMNHRVEITEGILADECAALLCDYYRMPRQVFNARKKVQSSINSGGSSDGGSSSETPGTSESATPESSGGSSGGSAKNTITKTLKLRIVRPYNSAEVEKIVADEKNNREKIALEKNKDKVKEACSEHLKVAAYCTTQVERNACLFCKARKLDDKFYQKLRGQFPDAVFWQEVGEIFRQLQKQAAEIYNQSLIELYYEILIKGKGIANASSVEHYLSDVCYTRAAELFKNAAIASGLRNKIKSNFRLKELRNMKSGLPTTKSDNFPIPLVRQKGGQYTGFEISNYNGDFIIKIPFGRWQVKKEINKYRPWEKFDFEQVRKSPKPISLLLSTQRRKRNKGWSKDEGTEAEIRKVMNGDYQTSYIEVKRGSKTGEKSAWMLNLSIDVPKIDKGVDPSIIGGIDVGVKSPLVCAINNAFSRYSISDNDLFRFNKKMFARRRILLKKNRHKRAGHGAKNKLKPISILTGKSERFRKKLIERWACEIADFFVKNKVGTVQMENLESMKRKEDSYFNIRLRGFWPYAEMQNRIEFKLKQYGIEIRKVAPNNTSKTCSKCGHLNNYFNFEYRKKNKFPHFKCEKCNFKENADYNAALNISNPMLKSTKEEP

SEQ ID NO: 341 - protein, 726 aa, synthetic construct
SEVEFSHEYWMRHALTLAKRARDEREVPVGAVLVLNNRVIGEGWNRAIGLHDPTAHAEIMALRQGGLVMQNYRLIDATLYVTFEPCVMCAGAMIHSRIGRVVFGVRNSKHGAAGSLVNVLNYPGMNHRVEITEGILADECAALLCDFYRMPRQVFNARKKAQPSINPGGSSGGSSGSETPGTSESATPESSGGSSGGSAKNTITKTLKLRIVRPYNSAEVEKIVADEKNNREKIALEKNKDKVKEACSKHLKVAAYCTTQVERNACLFCKARKLDDKFYQKLRGQFPDAVFWQEIGEIFRQLQKQAAEIYNQSLIELYYEIFIKGKGIANASSVEHYLSDVCYTRAAELFKNAAIASGLRNKVKSNFRLKELRSMKSGLPTTKSDNFPIPLVRQKGGQYTGFEISSHNDDFIIKIPFGRWQAKKEIDKYRPWEKFDFEQVRKSPKPISLLLSTQRRKRNKGWSKDEGTEAEIRKVMNGDYQTSYIEVKRGRKIGEKSVWMLNLSIDVPKIDKGVDPSTIGGIDVGVKSPLVCAINNAFSRYSISDNDLFRFNKKMFARRRILLKKNRHKRAGHGAKNKLKPITILTEKCGRFRKKLIERWACEIADFFIKNKVGTVQMENLESMKRKEDSYFNIRLRGFWPYAEMQNKIELKLKQYGIKIRKVAPNDTSKTCSKCGHLNDYFNFEYRKKNKFPHFKCEKCNFKEDADYNAALNISNPELKSTKEEP

SEQ ID NO: 342 - protein, 726 aa, synthetic construct
SEVEFSHEYWMRHALTLAKRARDEREVPVGAVLVLNNRVIGEGWNRAVGLHDPTAHAEIMALRQGGLVMQNYRLTDATLYVTFEPCVMCAGAMIHSRIGRVVFGVRNSKRGAAGSLMNVLNYPGMNHCVEITEGILMDECAALLCDFYRMPRQVLIAQKKAQSSISSGGSSGGSSCSETPGASESVTPKSSGGSSAGSTRNTITKTLKLRIVRPYNSAEVEKIVADEKNSREKIALEKNKDKVKEACSEHLKVAAYCTTQVERNACLFCKARKLDDRFYQKLRGQFPDAVFWQEIGEIFRQLQKQAAEIYNQSLIELYYEIFIKGKGFANASSVEHYLSDVCYTRAAELFKNAAIASGLRGKVKSNFRLKELKNMKSGLPTTKSDNFPIPLVKQKGGQYTGFEISNHNGDFIIKIPFGRWQVKKEISKHRPWEKFDFEQVRKSPKPISLLLSTQRRKRNKGWSKDEGTEAEIRKVMNGDYQTSYIEVKRGSKTGEKSAWMLNLSIDVPKIDKGVDPSIIGGIDVGVKSPLVCAINNALSRYSISDNDLFRFNKKMFARRRILLKKNRHKRAGHGARNKLKPITVLTEKSERFREKLIERWACEIANFFIKNKVGTVQMENLESMKRREDGYFNIRLRGFWPYAEMQSKIEFKLKQYGIEIRKVAPNNTSKTCSKCGHLNNYFNFEYRKKNKFPHFKCEKCNFKEDADYNAALNISNPKLKSTKEEP

SEQ ID NO: 343 - protein, 726 aa, synthetic construct
SEVEFSHEYWMRHALTLAKRARDEREVPVGAILVLNNRVIGEGWNRAIGLHDPTAHAEIMALRQGGLVMQNYRLIDATLYVTFEPCVMCAGAMIHSRIGRVVFGVRNSRHGAAGSLVNVLNYPGMNHRVEITEGILADECAALLCDFYRMPRQVFNARKKAQSSINPSGSSGGSSGSETPGTSESATPKSSGGSSGGPAKNTITKALKLRIVRPYNSAEVEKIVADEKNNRERIALEKNKDKVKEACSKHLKVAAYCTTQVERSACLFCKARKLDDRFYQKLRGQFPDAVFWQEIGEIFRQLQKQAAEVYNQSLVELYYEIFIKGKGITNASRVEHYLSDVCYTRAAELFKNAAIASGLRGKVKSNFRLKELKNMKSGLPTTKSDNFPIPLVKQKGGQYTGFEISSHNDDFIIKIPFGRWQVKKEIDKYRPWEKFDFEQVRKSPKPISLLLSTQRRKRNKGWSKDEGTEAEIRKVMNGDYQTSYIEVKRGSKTGEKSAWMLNLSIDVPKINKGVDPSIIGGIDVGVKSPLVCAINNAFSRYSISDNDLFRFNKKMFARRRILLGKNRHKRAGHGVKNKLKPITILTEKSGRFRKKLIERWACEIADFFVKNKVGTVQMENLESMKRKEDSYFNIRLRGFWPYAEMQNKIEFKLKQYGIKVRKVAPNNTSKTCSKCGHLNNYFNFEYRKKNKFPHFKCEKCNFKEDADYNAALNISNPKLKSTKEEP

SEQ ID NO: 344 - protein, 726 aa, synthetic construct
SEVEFSHEYWMRHALALAKRARDEREVPVGAVLVLNNRVIGEGWNRTTGLHDPTAHAEIMALRQGGLVMRNHRLTDATLYVTFEPCIMCAGAMIHSRIGRVVFGVRNSKRGAAGSLMNVLNYPGMNHCVEITEGILVDECAALLCDFYRMPRQVLNAQKKAQSSISPGGSSGGSSGSETPGASESVTPKSSGGSSGSSAKNTITKTLKLRIVRPYNSAEVEKIVADEKNNREKIALEKNKGKVKEACSKHLEVAAYCTTQVERNACPFCKARKLDDKFYQRLRGQFPDAVFWQELGEILRQLQKQAAEIYNQSLIELYYEIFIKGRGFANASSVEHYLSDVCYTRAAELFKNAAIASGLRGKVKSNFRLKELKNMKSGLPTTKSDNFPIPLVKQKGGQYTGFEISSHNDDFIIKIPFGRWQVKKEIDKYRPWEKFDFEQVRKSPKPISLLLSTQRRKRNKGWSKDEGTEAEIRKVMNGDYQTSYIEVKRGSKIGEKSAWMLSLSIDVPKIDKGVDPSIIGGIDVGVKSPLVCAINNAFNRYSISDNNLFHFNKKMFARRRILLKKNRHKRAGHGAKNKLKPISILTEKSERFRKKLIERWACEIADFFIRNKVGTVQMENLEGMKRREDSYFNIRLRGFWPYAEMQSKIEFKLKQYGIEVRKVAPNNTSKTCSKCGHLNNYFNFEYRKKNKFPHFKCEKCNFKEDADYNAALNISNPKLKSTKEEP

SEQ ID NO: 345 - protein, 726 aa, synthetic construct
SEVEFSHEYWMRHALTLAKRARDEREVPVGAVLVLNNRVIGEGWNRAIGLHDPTAHAEIMALRQGGLVMQNYRLIDATLYVTFEPCVMCAGAMIHSRIGRVVFGVRNSKHGAAGSLVNVLNYPGMNHRVEITEGILVDECAALLCDFYRMPRQVLNAQKKAQPSISSGGSSGGSSGSETPGTSESATPESSGGSSGGSAKNTITKTLTLRIVRPYNSAEVEKIVADEKNNREKIALEKNKDKVKEACSEHLKVATYCTTRVERNACPFCRARKLDDKFYQKLRGQFPDAVFWQELGEILRQLQKQAAEIYNQSLIELYYEIFIKGRGFANAGSVEHYLSDVCYTRAAELFKNAAIASGLRGKIKSNFRLKELKNMKSGLPTTKSDNFPIPLVKQKGGQYTGFEISSHNDDFIIKIPFGRWQVKKEIDKYRPWEKFDFEQVRKSPKPISLLLSTQRRKRNKGWSEDEGTEAEIRRVMNGDYQTSYIEVKRGSKIGEKSAWMLSLSIDVPKIDKGVDPSIIGGIDVGVKSPLVCAINNSFSRYSICDNDLFHFNKKMFARRRILLKKNRHKRAGHGAKNKLKPITILTGKSKRFRKKLIERWACEIAGFFIKNKVGTVQMENLESMKRREDSYFNIRLRGFWPYAEMQNKIEFKLKQYGIEIRKVAPNNTSKTCSRCGHLNNYFNFEYRKRNKFPHFKCEKCNFKENADYNAALNISNPKLKSPKEEP

SEQ ID NO: 346 - protein, 726 aa, synthetic construct
SEVEFSHEYWMRHALTLAKRARDEREVPVGAVLVLNDRVIGEGWNRTTGLHDPTAHAEIMALRQGGLVMQNYRLTDATLYVTFEPCVMCAGAMIHSRIGRVVFGVRNSKRGAAGSLMNVLNYPGMNHCVKITEGILVDECAALLCDFYRMPRQVLNAQKKAQSSISSGGSTGGSSGSETPGTSESPTPESSGGGSSGSAKNTITKTLQLRIVRPYNSAEVEKIVADEKSNREKIALEKNKDKVREACSKHLKVASYCTTQVERNACPFCKARKLDDKFYRKLRGQFPDAVFWQELGEILRQLQKQAAVIYNQSLIELYYEIFIKGKGITNASRVEHYLSDVCYTRAAELFKNAAIASGLRSKVRSNFRLKELKNMKSGLPTTKSDNFPIPLVKQKGGQYTGFEISSHNDDFIIKIPFGRWQVKKEIDKFRPWEKFDFEQVRKSPKPISLLLSTQRRKKNKGWSKDEGTEAEIRRVMNGDYQTSYIEVKRGSKIGGKSAWMLNLSIDVPKIDKGVDPSIIGGIDVGVKSPLVCAINNSSSRYSICDNDLFRFNKKMFARRRILLKKNRHKRAGHGAKNKLKPITILTKKSERFRKKLIERWVCEVADFFIKNKVGTVQMENLESMKRREDSYFNIRLRGFWPYAEMQNKIEFKLKQYGIEIRKVAPNDTSKTCSKCGHLNNYFNFEYRKKNKFPHFKCEKCNFKENADYNAALNISNPKLKSTKEEP

SEQ ID NO: 347 - protein, 726 aa, synthetic construct
SEVEFSHEYWMRHALSLAKRARDEREVPVGAVLVLNNRIIGEGWNRAIGLHDPTAHAEIMALRQGGLVMQNYRLIDATLYVTFEPCVMCAGAMIHSRIGRVVFGVRNNKHGAAGSLVNVLNCPGMNHRVEITEGILADECAALLCDFYRMPHQVFSARKKAQSSINPGGSSGGSSGSKTPGTSESATPESSGGSSGGSAKNSITKTLKLRIVRPYNSAEVEKIVADEKNNREKIALEKNKGKVKEACSKHLKVATYCTTQVERNACLFCKARKLDDKFYQKLRGQFPDAVFWQEIGEIFRQLQKQAAEIYNQSLIELYYEIFIKGKGFANASSVEHYLSDVCYTRAAELFKNAAIASGLRGKVKSNFRLKELKNMKSGLPTTKSDNFPIPLVKQKGGQYTGFEISSHNDDFIIKIPFGRWQVKKEIDKYRPWEKFDFEQVRKSPKPISLLLSTQRRKRNKGWSKDEGTEAEIRKVMNGDYQTSYIEVKRGSKIGEKSAWMLNLSIDVPRIDKGVDPSIIGGIDVGVKSPLICAINNAFSRYGISDNDLFRFNKKVFARRRILLKKNRHKRAGHGTKNKLKPITILTEKSGRFRKKLIERWACEIANFFIKNKVGTVQMENLESMKRKEDSYFNIRLRGFWPYAEMQNKIEFKLKQYGIKIRKVAPNNTSKTCSKCGHLNNYFSFEYRKKNKFPHFKCEKCNFKEDADYNAALNISNPKLKSTKGEP

SEQ ID NO: 348 - protein, 726 aa, synthetic construct; identical to SEQ ID NO: 336

SEQ ID NO: 349 - protein, 726 aa, synthetic construct
SEVEFSHEYWMRHALTLAKRARDEREVPVGAILVLNNRVIGEGWNRAIGLHDPTAHAEIMALRQGGLVMQNYRLIDATLYVTFEPCVMCAGAMIHSRIGRVVFGVRNSKHGAAGSLVNVLNYPGMNHRVEVTEGILADECAALLCDFYRMPRQVFNARKKAQSSINSGGSSGGSSGSETPGTSESATPKSSGGSSGGSAKNTITKTLKLRIVRPYNSAEVEKIVADEKSNREKIALEKNKDKVKEACSEHLKVAAYCTTQVERSACLFCKARKLDDKFYQKLRGQFPDAVFWQELGEILRQLQKQAAEIYNQSLIELYYEIFIKGRGFANASSVEHYLSDVCYTRAAELFKNAAIASGLRGKVKSNFRLKELKNMKSGLPTTKSDNFPIPLVKQKGGQYTGFEISSHNDDFIIKIPFGRWQAKKEIDKYRPWEKFDFEQVRKSPKPISLLLSTQRRKRNRGWSKDESTEAEIKRVMNGDYQTSYIEVKRGSKVGEKSAWMLNLSIDVPKIDKGVDPSIIGGIDVGVKSPLVCAINNALSRYSISDNDLFHFNKKMFARRRILLKKNKHKRAGHGTKNKLKPITILTEKSKRFRKKLIERWACEIADFFIKNKVGTVQMENLESMKRKEDSYFNIRLRGFWPYAEMQNKIEFKLKQYGIEIRKVAPNNTSKTCSKCGHLNSYFNFEYRKKNKFPHFKCEKCNFKENADYNAALNISNPKLKSTKEEP

SEQ ID NO: 350 - protein, 726 aa, synthetic construct
SEVEFSHEYWMRHALTLAKRARDEREVPVGAVLVLNNRVIGEGWNRAIGLHDPTAHAEIMALRQGGLVMQNYRLTDATLYVTFEPCVMCAGAMIHSRIGRVVFGVRNSKRGAAGSLMNVLNYPGMNHCVEVTEGILVDECAALLCDFYRMPRQVLNAQKKAQSSISSGGSSGGSSGSETPGASGSVTPKSSGGSSAGSTKDTITKTLKLRIVRPYNSAEVEKIVADEKNSREKIALEKNKDKVKEACSEHLKVAAYCTTQVERNACLFCKARKLDDGFYQKLRGQFPDAVFWQEIGEIFRQLQKQAAEIYNQSLIELYYEIFIKGKGFASASSVEHYLSDVCYTRAAELFKNAAIASGLRGKVKSNFRLKELKNMKSGLPTTKSDNFPIPLVKQKGGQYTGFEINSHNDDFIIKIPFGRWQVKKEIDKYRPWEKFDFEQVRKGPKPISLLLSTRRRKRNKGWSKDEGTEAEIRKVMNGDYQTSYIEVKRGSKIGEKSAWMLNLSIDVPKIDKGVDPSIVGGIDVGVKSPLVCAINNAFSRYSISDNDLFHFNKKMFARRRILLKKNRHKRAGHGAKNKLKPISILTEKSKRFRKKLIERWACEIADFFIKNKVGTVQMENLESMKRKEDSYFNIRLRGFWPYAEMQNKIEFKLKQYGIVVRKVAPNNTSKTCSECGHLNNYFNFEYRKKNKFPHFKCEKCNFKENADYNAALNISNPRLKSTKGEP

SEQ ID NO: 351 - protein, 726 aa, synthetic construct
SEVEFSHEYWMRYALTLAKRARDEREVPVGAVLVLNNRVIGVGWNRAIGLHDPTAHAEIMALRQGGLVMQNYRLIDATLYVTFEPCVMCAGAMVHSRIGRVVFGVRNSKRGAAGSLMNVLDYPGMDHRVEITEGILADECAALLCDFYRMPRQVFNAQKKAQSSISSGGSSGGSSGSETPGAGESVTPKSSVGSSAGSTKNTITKTLKLRIVRPYNSAEVEKIVADEKNNREKIALEKNKDKVKEACSKHLKVASYCTTQVERNACPFCKARKLDDKFYQKLRGQFPDAVFWQELGGIFRQLQKQAAEIYNQSLIELYYEIFIKGKGITNASRVEHYLSDVCYTRAAELFKNAAIASGLRSKVRSNFRLKELKNMKSGLPTTKSDNFPIPLVKQKGGQYTGFEISSHNSDFIIKIPFGRWQMKEEIDKYRPWEKFDFEQVRKSPKPISLLLSTQRRKRNKGWSKDEGTEAEIRKVMNGDYQTSYIEVKRGSKTGEKSTWMLNLSIDVPKIDKGVDPSIIGGIDVGVKSPLVCAINNAFSRYSISDNDLFRFNKKMFARRRILLKRNRHKRAGHGAKNKLKPISILTGKSERFRKKLIERWACEIADFFIKNKVGTVQMENLESMKRKEDSYFNIRLRGFWPYAEMQNKIEFKLKQYGIEIRKVAPNNTSKTCSKCGHLNNYFNFEYRKKNKFPHFKCEKCNFKENADYNAALNISNPKLKSTKEEP

SEQ ID NO: 352 - protein, 726 aa, synthetic construct
SEVEFSHEYWMRRALTLARRARDEREVPVGAVLVLNNRVIGEGWNRAIGLHDPTAHAEIMALRQGGLVMQNYRLVDATLYVTFEPCVLCAGAMVHSRIGRVVFGVRNSKRGAAGSLMNVLNYPGMNHRVEITEGILADECAALLCDFYRMPRQVFNARKKARSNINSSGSSGGSSGSETPGTSESATPESSGGSSGGSAKNTITKTLKLRIVRPYNSAEVEKIVADEKNNREKIALEKNKDKVKEACGKHLKVASYCTTQVERSACLFCKARKLDDKFYQKLRGQFPDAVFWQELGEIFRQLQKQAAEIYNQSLIELYYGIFIKGKGSANASSVEHYLSDVCYTRAAELFKNAAIASGLRGKVKSNFRLKELKNMKSGLPTTKSDNFPIPLVKQKGGQYTGFEISNHDDDFIIKIPFGRWQVKKEIDKYRPWEKFDFEQVRKSPKPISLLLSTQRRKRNKGWSKDEGTEAEIRKVMNGYYQTSYIEVKRGSKIGEKSAWMLNLSIDVPKIDKGVDPSIIGGIDVGVKSPLVCAINNAFSRYSISDNDLFRFNKKMFARRRILLKKNRHKRAGHGAKNKLKPITILTEKSKRFRRKLIERWACEIADFFIKNKVGTVQMENLESMKRKEDSYFNIRLRGFWPYAEMQNKIEFKLKQYGIEIRKVAPNNTSKTCSKCGHLNNYFNFEYRKMNKFPHFKCEKCNFKENADYNAALNISNPKLKSTKEEP

SEQ ID NO: 353 - protein, 726 aa, synthetic construct
SEVEFSHEYWMRHALTLAKRARDEREVPVGAILVLNNRVIGEGWNRAIGLHDPTAHAEIMALRQGGLVMQNYRLIDATLYVTFEPCVMCAGAMIHSRIGRVVFGVRNNKHGAAGSLVNVLNYPGMSHRVEITEGILADECAALLCDFYRMPRQVFNARKKAQSSIDPGGTSGGSSGSETPGTSECATPESSGGRSGGSAKNTITKTLKLRIVRPYNSTEVEKIVADEKNNREKIALEKNKDKVKEACSKHLKVASYCTTQVERNACLFCKARKLDDKFYQKLRGQFPDAVFWQELGGIFRQLQKQAAEIYNQSLIELYYEIFIKGKGITNASRVEHYLSDVCYTRAAELFKNAAIASGLRSKVRSNFRLKELKNMKSGLPTTKSDNFPIPLVKQKGGQYTGFEISSHNDDFIIKIPFGRWQVKKEIDKYRPWEKFDFEQVRKSPKPISLLLSTQRRKRNKGWSKDEGTEAEIRKVMNGDYRTSYIEVKRGSKIGEKSAWMLNLSIDVPKIDKGVDPSIIGGIDVGVKSPLVCAVNNSFSRYSICDNDLFRFNKKMFARRRILLKKNRHKRAGHGAKNKLKPITILTEKSKRFRKKLIERWACEIADFFIKNKVGTVQMENLESMKRKEDSYFNIRLRGFWPYAEMQNKIEFKLRQYGIVVRKVAPNNTSKTCSKCGHLNNYFNFEYRKKNKFPHFKCEKCNFKEVADYNAALNISNPKLKSTKEVP

SEQ ID NO: 354 - protein, 726 aa, synthetic construct
SEVEFNHEYWMRHALTLARRARDGREVPVGAVLVLNNRVIGEGWNRAIGLHDPTAHAEIMALRQGGLVMQNYRLIDATLYVTFEPCVMCAGAMVHSRIGRVVFGVRNSKRGAAGSLMNVLDYPGMNHRVEITEGILADECAALLCDFYRMPRQVFNAQKKAQSSINSGGSSGSSSGSETPGTSESATPESSGGSSGGSAKNTITKTLQLRIVRPYNSAEVEKIVTDEKNNREKIALEKNKDKVKEACSKHLKMAAYCTTQVERNACLFCKARRLDDKFYRKLRGQFSDAVFWQEIGEIFRQLQKQAAEIYNQSLIELYYEIFIKGKGITNASRVEHYLSDVCYTRAAELFKNAAIASGLRNKIKSNFRLKELKNMKSGLPTTKSDNFPIPLVKQKGGQYTGFEISSHNDDFIIKIPFGRWQVKEEIDKYRPWEKFDFEQVRKNPKPISLLLSTQRRKRNKGWSKDEGTEAEIRKVMNGDYQTSYIEVKRGSKIGEKSAWMLNLSIDVPKIDKGVDPSIIGGIDVGVKSPLVCAINNAFSRYSISDNDLFRFNKKVFARRRILLKKNRHKRAGHGTKNKLKPITILTEKSGRFRKKLIERWACEIANFFIKNKVGTVQMENLESMKRREDSYFNIRLRGFWPYAEMQSKIEFKLKQYGIKVRKVAPNNTSKTCSKCGHLNNYFSFEYRKKNKFPHFKCEKCSFKEDADYNAALNISNPKLKSPKEEP

SEQ ID NO: 355 - protein, 726 aa, synthetic construct
SEVEFSHEYWMRHALTLAKRARDEREVPVGAVLVLNNRVIGEGWNRAIGLQDPTAHAEIMALRQGGLVMQNYRLSDATLYVTFEPCVMCAGAMIHSRIGRVVFGVRNSKRGAAGSLMNVLNYPGMNHCVEITEGILVDECAALLCDFYRMPRQVLSAQKKAQSSVSSGGSSGGSSGSETPGASGSVTPKSSVGSSAGSTRNTITKTLKLRIVRPYNSAEVEKIVADEKNSREKIALEKNKDKVKEACSKHLKVAAYCTTQVERSACPFCKARKLDDKFYQKLRGQFPDAVFWQELGGIFRQLQKQAAEIYNQSLIELYYEIFIKGKGITNASRVEHYLSDVCYTRAAELFKNAAIASGLRSKVRSNFRLKELKNMKSGLPTTKSDNFPIPLVKQKGGQYTGFEISSHNSDFIIKIPFGRWQVKEEIDKYRPWEKFDFEQVRKGPKPISLLLSTQRRKRNKGWSKDEGTEAEIRKVMNGDYQTSYIEVKRGSRIGEKSAWMLSLSIDVPKIDKGVDPSIIGGIDVGVKSPLVCAINNAFSRYSISDNDLFRYNKKMFARRRILLKKNRHKRAGHGARNKLKPISILTEKSKRYRKKLIERWACEIADFFIKNKVGTVQIENLESMKRREDSYFNIRLRGFWPYAEMQNKIEFKLKQYGIEIRKVAPNNTSKTCSKCGHLNSYFNFEYRRKNKFPHFKCEKCNFKEDADYNAALNISNPKLKSTKEEP

SEQ ID NO: 356 - protein, 726 aa, synthetic construct
SEVEFSHEYWMRRALTLAKRARDGCEVPVGAVLVLNNRVIGEGWNRAIGLHDPTAHAEIMALRQGGLVLQNYRLIDATLYVTFEPCVMCAGAMIHSRIGRVVFGVRNNKHGAAGSLVNVLNYPGMNHRVEITEGILADECAALLCDFYRMPRLVFNARKKTQSSINPGGSSGGSSGSETPGTSESATPESSGGSSGGSAKNTITKTLKLRIVRPYNSAEVEKIVADEKNNREKIALEKNKDKVKEACSKHLKMASYCTTQVERNACLFCKARKLDDKFYQKLRGQFPDAVFWQELGGIFRQLQKQAAEIYNQSLIELYYEIFIKGKGITNASRVEHYLSDVCYTRAAELFKNAAIASGLRNKIKSNFRLKELRNMKSGLPTTKSDNFPIPLVKQKGGQYTGFEISSHNDDFIIKIPFGRWQVKKEIDKYRPWEKFDFEQVRKSPKPISLLLSTQRRKRNKGWSKDEGTEAEIRKVMNGDYQTSYIEVKRGSKTGEKSAWMLNLSIDVPKIDKGVDPSIIGGIDVGVKSPLVCAINNALSRYSISDNDLFHFNKKMFARRRILLRKNRHKRAGHGAKNKLKPITIMTEKSKRFRKKLIERWACEIADFFIKNKVGTVQMENLESMKRKEDSYFNIRLRGFWPYAEMQNKIEFKLRQYGIEVRKVAPNNTSKTCSKCGHLNNYFNFEYRKKNKFPHFKCEKCNFKEDADYNAALNISSPKLKSTKGEP

SEQ ID NO: 357 - protein, 726 aa, synthetic construct
SEVEFSHEHWMRHALTLAKRARDEREVPVGAVLVLNNRVIGEGWNRAIGLHDPTAHAEIMALRQGGLVMQNYRLTDATLYVTFEPCVMCAGAMIHSRIGRVVFGVRNSKRGAAGSLMNVLNYPGMNHCVEITEGILVDECAALLCDYYRMPRQVLSAQKKARSSISSGGSSGGSSGSETPGASGSVTPKSSVGSSAGSTKNTITKTLKLRIVRPYNSAEVEKIVADEKNNREKIALEKNKGKVKEACSKHLEVAAYCTTQVERNACLFCKARKLDDKFYQKLRDQFPDAVFWQELGEIFRQLQKQAAEIYNQSLIELYYEIFIKGKGFANASNVEHYLSDVCYTRAAELFKNAAIASGLRGKVKSNFRLKELKNMKSGLPTTKSDNFPIPLVKQKGGQYTGFEISSHNDDFIIKIPFGRWQVRKEIDKYRPWEKFNFEQVRKSPKPISLLLSTQRRKRNKGWSKDEGTEAEIRKVMNGDYQTSYIEVKRGSKIGEKSAWMLCLSIDVPKIDKGVDPSIIGGIDVGVKSPLVCAINNAFNRYSISDNNLFHFNKKMFARRRILLKKNRHKRAGHGVKNKLKPISILTEKSERFRKKLIERWACEIADFFIRNKVGTVQMENLEGMKRKEDSYFNIRLRGFWPYAEMQNKIEFKLKQYGIVVRKVAPNDTSKTCSKCGHLNNYFNFEYRKKNKFPHFKCEKCNFKENADYNAALNISNPKLKSTKGEP

SEQ ID NO: 358 - protein, 726 aa, synthetic construct
SEVEFSHEYWMRHALTLAKRARDEREVPVGAILVLNNRVIGEGWNRAIGLHDPTAHAEIMALRQGGLVMQNYRLIDATLYVTFEPCVMCAGAMIHSRIGRVVFGVRNNKHGAAGSLVNVLNYPGMNHRVEITEGILADECAALLCDFYRMPRQVFNARKKARSNINSGGSSGGSSGSETPGTSESAAPESSGGSSGGSTRNTITKTLKLRIVRPYNSAEVEKIVADEKNNREKIALEKNRDKVKEACSKHLKVAAYCTTQVERNACLFCKARKLDDKFYQKLRGQFPDAVFWQEISEIFRQLQKQAAEIYNQSLIELYYEILIKGKGFANASSVEHYLSDVCYTRAAELFKNAAIASGLRGKVKSNFRLKELKNMRSGLPTTKSDNFPIPLVKQKGGQYTGFEINSHNDDFIIKIPFGRWQVKKEIDKYRPWEKFDFEQVRKSPKPISLLLSTQRRKRNKGWSKDEGTEAEIRKVMNGDYQTSYIEVKRGSKTGEKSAWMLNLSIDVPKIDKGVDPSIIGGIDVGVKSPLVCAINNAFSRYSISDNDLFRFNKKMFARRRILLKKNRHKRAGHGAKNKLKPISILTGKSERFRKKLIERWACEIADFFIKNKVGTVQMENLESMKRKEDSYFNIRLRGFWPYAEMQNKIEFKLKQYGIEIRKVAPNNTSKTCSKCGHLNNYFNFEYRKMNKFPHFKCEKCNFKENADYNAALNISNPKLKSTKEEP

SEQ ID NO: 359 - protein, 726 aa, synthetic construct
SEVEFSHEYWMRHALTLAKRARDEREVPVGAILVLNNRVIGEGWNRAIGLHDPTAHAEIMALRQGGLVMQNYRLTDATLYVTFEPCVMCAGAMIHSRIGRVVFGVRNNKHGAAGSLVNVLNYPGMNHRVETTEGILADECAALLCDFYRMPRRVFNARKKAQSSISPGGSSGGSSGSETPGTSESATPESSGGSSGGSAKNTITKTLKLRIVRPYNSAEVEKIVADEKNSREKIALEKNKDKVKEACSKHLKVAAYCTTQVERNACPFCKARKLDDKFYQKLRGQFPDAVFWQELGEIFRQLQKQAAEIYNQSLIELYYEIFIKGRGFANAGSVEHYLSDVCYTRAAELFKNAAIASGLRGKVKSNFRLKELKNMKSGLPTTKSDNFPIPLVKQKGGQYTGFEISSHNDDFIIKIPFGRWQVKKEIDKYRPWEKFDFEQVRKSPKPISLLLSTKRRKRSKGWSKDEGTEAEIRKVMNGDYQTSYIEVKRGSKAGEKSAWMLSLSIDVPKIDKGVDPSIIGGIDVGVKSPLVCAINNALSRYSISDNDLFHFNKKMFARRRILLKKNKHKRAGHGARNKLKPITVLTEKSERFRKKLIERWACEVANFFIKNKVGTVQMENLESMKRKEDSYFNIRLRGFWPYAEMQNKIEFKLKQYGIEIRKVAPNNTSKTCSKCGHLNNYFNFEYRKTNKFPYFKCEKCNFKEDADYNAALNISNPKLKSTKEEP

SEQ ID NO: 360 - protein, 726 aa, synthetic construct
SEVEFSHEYWMRHALTLAKRARDEREVPVGAILVLNNRVIGEGWNRAIGLHDPTAHAEVMALRQGGLVMQNYRLIDATLYVTFEPCVMCAGAMIHSRIGRVVFGVRNSKHGAAGSLMNVLNYPGMNHRVEITEGILADECAALLCDFYRMPRQVFNARKKAQSSINPGGPSGGSSGSETPDTSESATPESSGGNSGGSAKNTITKTLKLRIVRPYNSAEVEKIVADEKNNREKIALEKNKDKVKEACSEHLKVAAYCTTQVERNACLFCKARKLDDKFYQKLRGQFPDAVFWQEIGEIFRQLQKQAAEIYNQSLIELYYEIFIKGKGFANASSVEHYLSDVCYTRAAELFKNAAIASGLRGKVKSNFRLKELKNMKSGLPTTKSDNFPIPLVKQKGGQYTGFEISSHNDDFIIKIPFGRWQVKKEIDKYRPWEKFDFEQVRKSPKPISLLLSTQRRKRNKGWSKDEGTEAEIRKVMNGDYQTSYIEVKRGSKTGEKSAWMLNLSIDVPKIDKGVDPSTIGGIDVGVKSPLVCAINDAFSRYSISDNDLFRFNKKMFARRRILLKKNRHKRAGHGAKNKLKPITILTEKSKRFRKKLIERWACEIADFFIKNKVGTVQMENLESMKRKEDSYFNIRLRGFWPYAEMQNKIEFKLKQYGIEVRRVAPNNTSKTCSKCGHLNNYFNFEYRKKNKFPHFKCEKCNFKENADYNAALNISNPKLKSTKEKP

SEQ ID NO: 361 - protein, 726 aa, synthetic construct
SEVEFSHEYWMRHALTLAKRARDEREVPVGAILVLNNRVIGEGWNRAIGLHDPTAHAEIMALRQGGLVMQNYRLTDATLYVTFEPCVMCAGAMIHSRIGRVVFGVRNSKRGAAGSLMNVLNYPGMNHCVEITEGILVDECAALLCDFYRMPRQVLNAQKKAQPSISSGGSSGGCSGSEMPGASESVTPKSSGGSSAGSTKNTITKTLKLRIVRPYNSAEVEKIVADEKNSREKIALEKNKDKVKEACSEHLKVAAYCTTQVERNACLFCKARKLDDKFYQKLRGQFPDAVFWQELGGIFRQLQKQAAEIYNQSLIELYYEIFIKGKGITNASRVEHYLSDVCYTRAAELFKNAAIASGLRGKVKSNFRLKELKNMKSGLPTTKSDNFPIPLVKQKGGQYTGFEISSHNDDFIIKIPFGRWQVKEEIDKYRPWEKFDFEQVRKDPKPISLLLSTQRRKRNKGWSKDEGTEAEIRRVMNGDYQTSYIEVKRGSKIGEKSAWMLNLSIDVPKIDKGVNPSIIGGIDVGVKSPLVCAINNSSSRYSISDNDLFHFNKKMFARRRILLKKNRRKRAGHGAKNKLKPITILTEKSGRFRKKLIERWACEIADFFIKNKVGTVQMENLESMKRKEDSYFNIRLRGFWPYAEMQNRIEFKLKQYGIEIRKVAPNNTSKTCSKCGHLNNYFNFEYRKKNKFPHFKCEKCNFKENADYNAALNISNPRLKSTKEEP

SEQ ID NO: 362 - protein, 726 aa, synthetic construct
SEVEFSHEYWMRHALTLAKRARDEREVPVGAVLVLNNRAIGEGWNRAIGLHDPTAHAEIMALRQGGLVMQNYRLTDATLYVTFEPCVMCAGAMIHSRIGRVVFGVRNSKRGAAGSLMNVLNYPGMNHCVEITEGILADECAALLCDFYRMPRQVFNARKKAQSSINSGGSSGGSSGSETPGTSESATPKNSGGSSGGSAKNTITKALKLKIVRPYNSAEVEKIVADEKNNRERIALEKNKDKVKEACSKHLKVAAYCTTQVERNACLFCKARKLDDKFYQKLRGQFPDAVFWQEIGEIFRQLQKQAAEIYNQSLIELYYEIFIKGKGITNASRVEHYLSDVCYTRAAELFKNAAIASGLRSKVRSNFRLKELKNMKSGLPTTKSDNFPIPLVKQKGGQYTGFEISSHNSDFIIKIPFGRWQVKEEIDKYRPWEKFDFEQVRKSPKPISLLLSTQRRKKNKGWSKDEGTEAEIRRVMNGDYQTSYIEVKRGSKIGEKSAWMLNLSIDVPKIDKGVDPSIIGGIDVGVKSPLVCAINNSSSRYSICDNDLFRFNKKMFARRRILLKKNRHKRAGHGAKNKLKPITILTKKSERFRKKLIERWVCEVADFFIKNKVGTVQMENLESMKRKEDSYFNIRLRGFWPYAEMQNKIEFKLKQYGIEIRKVAPNNTSKTCSKCGHLNNYFNFEYRKKNKFPHFKCEKCNFKEDADYNAALNISNPKLKGTKEEP

SEQ ID NO: 363 - protein, 726 aa, synthetic construct
SEVEFSHEYWMRHALTLAKRARDEREVPVGAILVLNNRVIGEGWNRAIGLHDPTAHAEIMALRQGGLVMQNYRLIDATLYVTFEPCVMCAGAMIHSRIGRVVFGVRNNKHGAAGSLVNVLDYPGMNHRVEITEGILADECAALLCDFYRMPRQVFNARKKAQSSINPGGSSGGSSGSETLGTSENATPESSGGSSGSSAKNTITKTLKLRIVRPYNSAEVEKIVADEKNNREKIALEKNKDKVKEACSKHLKVAAYCTTQVERNACLFCKARRLDDKFYQKLRGQFPDAVFWQEIGEIFRQLQKQAAEIYNQSLVELYYEILIKGKGIANASSVEHYLSDVCYTRAAKLFKNAAIASGLRNKIKSNFRLKELRNMKSGLPTTKSDNFPIPLVKQKGGQYTGFEISNHNSDFIIKIPFGRWQAKKEIDRYRPWEKFDFEQVRKNPKPISLLLSTRRRERNKGWSKDEGTEAEIRRVMNGDYQTSYIEVKRGSKIGEKGAWMLSLSIDVPKIDKGVDPRIIGGIDVGVKSPLVCAINNVLSRYSISDNDLFHFNKKMFARRRILLKKNGHKRAGHGAKNKLKPITIMTEKSKRFRKKLIERWACEIADFFIKNKVGTVQMENLESMKRKEDSYFNIRLRGFWPYAEMQNKIEFKLKQYGIVVRKVAPNNTSKTCSKCGHLNNYFNFEYRKKNKFPHFKCEKCNFKEDADYNAALNISNPKLKSTKGEP

SEQ ID NO: 364 - protein, 726 aa, synthetic construct
SEVEFSHEYWMRHALSLAKRARDEHEVPVGAVLVLNNRIIGEGWNRAIGLHDPTAHAEIMALRQGGLVMQNYRLTDATLYVTFEPCVMCAGAMVHSRIGRVVFGVRNSKRGAAGSLMNVLNYPGVNHCVEITEGILVDECAALLCDFYRMPRQVLNAQKKAQSSISSGGPSGGCSGSEMPGASGSVTPKSSGGSSAGSTKNTITKTLKLRIVRPYNSAEVEKIVADEKNSREKIALERNKDKVKEACSEHLKVAAYCTTQVERNACLFCKARKLDDRFYQKLRGQFPDAVFWQETGEIFRQLQRQAAEIYNQSLIELYYEIFIKGKGFANASSVEHYLSDVCYTRAAELFKNAAIASGLRGKVKSNFRLKELKNMKSGLPTTKSDNFPIPLVKQKGGQYTGFEISSHNDDFIIKIPFGRWQVKKEIDRYRPWEKFDFEQVRKSPKPISLLLSTQRRKRNKGWSKDEGTEAEIRKVMNGDYQTSYIEVKRGSKTGEKSAWMLNLSIDVPKIDKGVDPSIIGGIDVGVKSPLVCAINNAFSRYSISDNDLFRFNKKMFARRRILLKKNRHKRAGHGAKNKLKPISILTGKSERYRKKLIERWACEIADFFIKNKVGTVQMENLESMKRKEDSYFNIRLRGFWPYAEMQNKIEFKLKQYGIEIRKVAPNNTSKTCSKCGHLNNYFSFEYRKKNKFPHFKCEKCNFREDADYNAALNISNPKLKSTKEDL

SEQ ID NO: 365 - protein, 726 aa, synthetic construct
SEVEFSHEYWMRHALILAERARDEREVPVGAVLVLNNRVIGEGWNRAIGLHDPTAHAEIMALRQGGLVMQNYRLIDATLYVTFEPCVMCAGAMIHSRIGRVVFGVRNSKRGAAGSLMNVLNYPGMNHRVEITEGILTDECAALLCDFYRMPHQVLNAQKKAQSSINSGGSSGSSSGSETPGTGGSATPEGSGSSSGGFAKGTITKTLKLRIVRPYNSAEVEKIVADEKNNREKIALEKNKGKVKEACSKHLKVATYCTTQVGRNACLFCKARKLDDKFYQKLRGQFPDAVFWQEIGEIFRQLQKQAAEIYNQSLIELYYEIFIKGKGSANASSVEHYLSDVCYTRAAEQFKNAAIASGLRGKVKSNFRLKELKNMKSGLPTTKSDNFPIPLVKQKGGQYTGFEISNHNGDFIIKIPFGRWQAKKEIDKYRPWEKFDFEQVRKSPKPISLLLSTQRRKKNRGWSRDEGTEAEIKKVMNGDYQTSYIEVKRGSKIGEKSAWMLNLSIDVPKIDKGVDPSIIGGIDVGVKSPLVCAINNAFSRYSISDNDLFRFNKKMFARRRILLKKNRHKRVGHGAKNKLKPISILTGKSERFRKKLIERWACEIADFFIKNKVGTVQMENLESMKRKEDSYFNIRLRGFWPYAEMQNKIEFKLKQYGIKVRKVAPNNTSKTCSKCGHLNNYFSFEYRKKNKFPHFKCEKCNFKENADYNAALNISNPKLKGTKEEP

SEQ ID NO: 366 - protein, 726 aa, synthetic construct
SEVEFGHEYWMRHALTLAKRARDEREVPVGAVLVLNNRVIGEGWNRAIGLHDPTAHAEIMALRQGGLVMQNHRLVDATLYVTFEPCVLCAGAMIHSRIGRVVFGVRNSKRGAAGSLMNVLNYPGMNHRVEITEGILADECTALLCDYYRMPRQVFNARKKAQSSINSGGSSDGGSGSETPGTSESATPESSGGSSGGSAKNTITKTLKLRIVRPYNSAEVEKIVADEKNNREKIALEKNKDKVKEACSEHLKVAAYCTTQVERSACLFCKARKLDDKFYQKLRGQFPDAVFWQEIGEIFRQLQKQAAEIYNQSLIELYYEIFIKGKGFANAGSVEHYLSDVCYTRAAELFKNAAIASGLRGKVKSNFRLKELKNMRSGLPTTKSDNFPIPLVKQKGGQYTGFEISSHNDDFIIKIPFGRWQVKEEIDKYRPWEKFDFEQVRKNPKPISLLLSTQRRKRNKGWSKDEGTEAEIRKVMNGDYQTSYIEVKRGSKIGEKSAWMLNLSIDVPKIDKGVDPSIIGGIDVGVKSPLVCAINNAFSRHSISDNDLFHFNKKMFARRRILLKKNRHKRAGHGAKNKLKPISILTEKSKRFRKKLIERWACEIADFFIKNKVGTVQMENLESMKRKEDSYFNIRLRGFWPYAEMQNKIEFKLKQYGIEIRKVAPNNTSKTCSKCGHLNNYFNFEYRKKNKFPHFKCEKCNFKENADYNAALNISNPKLKSTKEEP

SEQ ID NO: 367 - protein, 726 aa, synthetic construct
SEVEFSHEYWMRHALTLAKRARDEREVPVGAVLVLNNRVIGEGWNRAIGLHDPTAHAEIMALRQGGLVMQNYRLTDATLYVTFEPCVMCAGAMIHSRIGRVVFGVRNSKRGAAGSLMNVLNYPGMNHCVEITEGILVDECAALLCDFYRMPRQVLNAQKKAQSSISSGGSSGSSSGSETPGASESVTPKSSVGSSAGSTKNTITKTLKLRIVRPYNSAEVEKIVADEKNNREKIALEKNKDKVKEACSKHLKVAAYCTTQVERNACPFCKARRLDDKFYQKLRGQFPDAVFWQEIGEIFRQLQKQAAETYNQSLIELYYEIFIKGKGFANASSVEHYLSDVCYTRAAELFKNAAIASGLRGKVKSNFRLKELKNMKSGLPTTKSDNFPIPLVKQKGGQYTGFEISSHNDDFIIKIPFGRWQVKKEIDKYRPWEKFDFEQVRKSPKPISLLLSTQRRKRNKGWSKDEGTEAEIRKVMNGDYQTSYIEVKRGSKTGEKSAWMLNLSIDVPKIDKGVDPCIIGGIDVGVKSPLVCAINNAFSRYSISDNDLFHFNRKMFARRRILLKKNGHKRAGHGARNKLKPITIMTEKSKRFRKKLIERWACEIADFFIKNKVGTVQMENLESMKRKEDSYFNIRLRGFWPYAEMQNKIEFKLKQYGIVVRKVAPNNTSKTCSKCGHLNNHFNFEYRKKNKFPHFKCEKCNFKEDADYNAALNISNPKLKSTKEEP

SEQ ID NO: 368 - protein, 726 aa, synthetic construct
SEVEFSHEYWMRHALTLAKRARDEREVPVGAILVLNNRVIGEGWNRAIGLHDPTAHAEIMALRQGGLVMQNYRLIDATLYVTFEPCVMCAGAMIHSRIGRVVFGVRNSKHGAAGSLVNVLNYPGMNHRVEITEGILADECAALLCDFYRMPHQVFGARRKAQSSINPGGSSGGSSGSETPGASESVTPKSSVGSSAGSTKNTITKTLKLRIVRPYNSAEVEKIVADEKDNRERIALERNKDKVKEACSEHLKVAAYCTTQVERNACLFCKARKLDDRFYQKLRGQFPDAVFWQETGEIFRQLQRQAAEIYNQSLIELYYEIFIKGKGFANASSVEHYLSDVCYTRAAELFKNAAIASGLRGKVKSNFRLKELKNMKSGLPTTKSDNFPIPLVKQKGGQYTGFEISSHNDDFIIKIPFGRWQVKKEIDKYRPWEKFDFEQVRKSPKPISLLLSTQRRRRNKGWSKDEGTEAEIRKVMNGDYQTSYIEVRRGSKIGEKSAWMLSLSIDVPKIDKGVDPSIIGGIDVGVKSPLVCAINNAFCRYSISDNDLFHFNKKMFARRRILLKKSRHKRAGHGAKNKLKPISILTEKSERFRKKLIERWACEIADFFIKNKVGTVQMENLESMKRREDSYFNIRLRGFWPYAKMQNKIEFKLKQYGIEIRKVAPNNTSKTCSKCGHLNNYFNFEYRKKNKFPHFKCEKCNFKENADYNAALNISNPKLKSTKGEP

SEQ ID NO: 369 - protein, 726 aa, synthetic construct
SEVEFSHEYWMRRALTLAKRARDEREVPVGAVLVLNNRVIGEGWNRAIGLHDPTAHAEIMALRQGGLVMQNYRLIDATLYVTFEPCVMCAGAMVHSRIGRVVFGVRNSKRGAAGSLMNVLDYPGMGHRVEITEGILADECAALLCDFYCMPRQVFNAQKRAQSSINSGGSSGGSSDSETPGTSESATPESSGGGSSGSAKDTITKTLQLRIVRPYNSAEVEKIVADEKNNREKIALEKNKDKVKEACSKHLKVASYCTTQVERNACPFCKARKLDDKFYQKLRGQFPDAMFWQELGEILRQLQKQAAEIYNQSLIELYYEIFIKGKGFANASSVEHYLSDVCYTRAAELFKNAAIASGLRGKVKSNFRLKELKNMKSGLPTTKSDNFPIPLVKQKGGQYAGFEISSHNDDFIIKIPFGRWQAKKEIDKYRPWEKFDFEQVRKSPKPISLLLSTQRRKKNKGWSKDEGTEAEIRKVMNGGYQTSYIEVKRGSKIGEKSAWMLNLSIDVPKIDKGVDPSIIGGIDVGVKSPLVCAINNAFSRYSISDNDLFRFNKKMFARRRILLKKNRHKRAGHGAKNKLKPISILTEKSKRFRKKLIERWACEIADFFIKNKVGTVQMENLESMKRKEDSYFNIRLRGFWPYAEMQNKIEFKLKQYGIEIRKVAPNNTSKTCSKCGHLNNYFNFEYRKKNKFPHFKCEKCNFKENADYNAALNISNPKLKSTKGEP

SEQ ID NO: 370 - protein, 726 aa, synthetic construct
SEVEFSHEYWMRHALTLAKRARDEHEVPVGAVLVLNNRVIGEGWNRAIGLHDPTAHAEIMALRQGGLVMQNYRLTDATLYVTFEPCVMCAGAMIHSRIGRVVFGVRNSKRGAAGSLMNVLNYPGMNHCVEITEGILVDECAALLCDFYRMPRQVLNAQKKAQSSISSGGSSGGCSGSEMPGASESVTPKSSGGSSAGSTKNTITKTLKLRIVRPYNSAEVEKIVADEKNSREKIALERNKDKVKEACSEHLKVATYCTTQVERNACLFCKARKLDDRFYQKLRGQFPDAVFWQETGEIFRQLQRQAAEIYNRSLIELYYEIFIKGKGFANASSVEHYLSDVCYTRAAELFKNAAIASGLRGKVKSNFRLKELKNMKSGLPTTKSDNFPIPLVKQKGGQYTGFEISSHNDDFIIKIPFGRWQVKKEIDKYRPWEKFDFEQVRKSPKPISLLLSTQRRKRNKGWSKDEGTEAEIRRVMNGDCQTSYIEVKRGSKIGEKSAWMLNLSIDVPKIDKGVDPSIIGGIDVGVKSPLVCAINNAFSRYSISDNDLFHFNKKMFARRRILLKKTRHKRAGHGAKNKLKPISILTEKSERFRKKLIERWACEIADFFIKNKVGTVQMENLESMKRREDSYFNIRLRGFWPYAKMQNKIEFKLKQYGIKVRKVAPNNTSKTCSKCGHLNNYFSFEYRKKNKFPHFKCEKCNFKENADYNAALNISNPKLKSTKEEP

SEQ ID NO: 371 - protein, 726 aa, synthetic construct
SEVEFSHEYWMRHALTLAKRARDEREVPVGAILVLNNRVIGVGWNRAIGLHDPTAHAEIMALRQGGLVMQNYRLIDATLYVTFEPCVMCAGAMIHSRIGRVVFGVRNSKHGAAGSLVNVLNYPGMNHRVEITEGILADECAALLCDFYRMPRQVFNARKKAQSSINSGGSSGGSSGSETPGTSESATPKSSGGSSGGSAKNTITKALKLRIVRPYNSAEVEKIVADEKNNRERIALEKNKDKVKEACSKHLKVAAYCTTQVERNACLFCKARKLDNKFYQKLRGQFPDAVFWQEIGEIFRQLQKQAAEIYNQSLIELYYEIFIKGKGFANASSVEHYLSDVCYARAAELFKNAAIASGLRGKVKSNFRLKELKNMRSGLPTTKSDNFPIPLVRQKGGQYTGFEISSHNDDFIIKIPFGRWQAKKEIDKYRPWEKFDFEQVRKSPKPISLLLSTQRRKRNKGWSKDEGTEAEIRKVMNGDYQTSYIEVKRGSKTGEKSAWMLNLSIDVPKIDKGVDPCIIGGIDVGVKSPLVCAINNAFSRYSISDNDLFRFNKKMFARRRILLKKNRHKRAGHGAKNKLKPISILTRKSERFRRKLIERWACEIADFFIKNKVGTVQMENLESMKRKEDSYFNIRLRGFWPYAEMQNKIEFKLKQYGIEIRKVAPNNTSKTCSKCGHLNNYFSFEYRKRNKFPHFKCEKCNFKEDADYNAALNISNPKLKSTKEEP

SEQ ID NO: 372 - protein, 726 aa, synthetic construct
SEVEFSHEYWMRHALSLAKRARDEREVPVGAVLVLNNRIIGEGWNRAIGLHDPTAHAEIMALRQGGLVMQNNRLTDATLYVTFEPCVMCAGAMVHSRIGRVVFGVRNSKRGAAGSLMNVLNYPGVNHCVEITEGILVDECAALLCDFYRMPRHVLNAQKKAQSSINSGGSSGGSSGSETPGTGGSATPEGSGGSSGGFAKSTITKTLKLRIVRPYNSAEVEKIVADEKNNREKIALEKNKDKVKEACSEHLKVAAYCTTQVERSACLFCKARKLDDKFYQKLRGQFPDAVFWQELGGIFRQLQKQAAEIYNQSLIELYYEIFIKGKGITNASRVEHYLSDVCYTRAAELFKNAAIASGLRSKVRSNFRLKELKNMKSGLPTTKSDNFPIPLVKQKGGQYTGFEISSHNDDFIIKIPFGRWQVKKEINKYRPWEKFDFEQVRKSPKPISLLLSTQRRKRNKGWSKDEGTEAEIRKVMNGDYQTSYIEVKRGSKIGEKSAWMLNLSIDVPKIDKGVDPSIIGGIDVGVKSPLVCAINNAFSRFSISDNDLFHFNKKMFARRRILLKKNRHKRAGHGAKNKLKPISILTGKSERFRKKLIERWACEIADFFIKNKVGTVQMENLEGMKRKEDSYFNIRLRGLWPYAEMQNKIEFKLKQYGIEIRKVAPNNTSKTCSKCGHLNNYFNFEYRKKNKFPHFKCEKCNFKENADYNAALNISNPKLKNTKEEP

SEQ ID NO: 373 - protein, 726 aa, synthetic construct
SEVEFSHEYWMRHALTLAKRARDEREVPVGAVLVLNNRVIGEGWNRAIGLHDPTAHAEIMALRQGGLAMQNYRLVDATLYVTFEPCVLCAGAMVHSRIGRVVFGVRNSKRGAAGSLMNVLNHPGMNHRVEITGGILADECAALLCDFYRMPRQVFNAQKKARSNINSGGPSGGSSGSETLGTSESATPESSGGSSGGSAKNTITKTLKLRIVRPYNSAEVEKIVADEKNSREKIALERNKDQVKEACSKHLEVAAYCTTQVERNACLFCKARKLDDKFYQKLRGQFPDAVFWQELGEIFRQLQKQAAEIYNQSLIELYYEIFIKGKGFANAGSVEHYLSDVCYTRAAELFKNAAIASGLRNKIKSNFRLKELRNMRSGLPTTKSDNFPIPLVRQKGGQYTGFEISNHDGDFIIKIPFGRWQVKKEINKHRPWEKFDFEQVRKSPKPISLLLSTQRRKRNKGWSKDEGTEAEIRKVMNGDYQTSYIEVKRGSKIGEKSAWMLNLSIDVPKIDKGVDPGIIGGIDVGVKSPLVCAINNASSRYSISDNDLFHFNKKMFARRRILLRKNRHKRAGHGAKNKLKPITIMTEKSKRFRKKLIERWACEIADFFIKNKVGTVQMENLESMKRKEDSYFNIRLRGFWPYAEMQNKIEFKLKQYGIEIRKVAPNNTSKTCSKCGHLNNYFNFEYRKKNKFPHFKCEKCNFKENADYNAALNISNPKLKSTKEEP

SEQ ID NO: 374 - protein, 726 aa, synthetic construct
SEVEFSHEYWMRRALTLAKRARDEREVPVGAVLVLNNRVIGVGWNRAVGLHDPTAHAEIMALRQGGLVMQNYRLFDATLYVTFEPCVMCAGAMIHSRIGRVVFGVRNSKRGAAGSLMNVLNYPGMNHCVEITEGILVDECAALLCDFYRMPRQVLSAQKKAQSSVSSGGSSGGSSGSETPGTSGSVTPKSSVGSSAGSTKNTITKTLKLRIVRPYNSAEVEKIVADEKNNREKIALEKNKDKVKEACSKHLKVAAYCTTQVERNACLFCKARKLDDKFYQKLRGQFPDAVFWQEIGEIFRQLQKQAAEIYNQSLIELYYEIFIKGKGFANASSVEHYLSDVCYTRAAELFKNAAIASGLRGKVKSNFRLKELKNMKSGLPTTKSDNFPIPLVKQKGGQYTGFEISSHNDDFIIKIPFGRWQVKKEIDKYRPWEKFDFEQVRKSPKPISLLLSTQRRKRNKGWSKDEGTEAEIRKVMNGDYQTSYIEVKRGSKTGEKSAWMLNLSIDVPKIDKGVDPSIIGGIDVGVKSPLVCAINNAFSRYSISDNDLFRFNKKMFARRRILLKKNGHKRAGHGAKNKLKPISILTEKSKRFRKKLIERWACEIADFFIKNKVGTVQMENLESMKRKEDSYFNIRLRGFWPYAEMQNRIEFKLKQYGIEIRRVAPNNTSRTCSKCGHLNNYFNFEYRKKNKFPHFKCEKCNFREDADYNAALNISNPKLKSTKEEP

SEQ ID NO: 375 - protein, 726 aa, synthetic construct
SEVEFSHEYWMRHALTLAKRARDEREVPVGAVLVLNNRVIGEGWNRAIGLHDPTAHAEIMALRQGGLVMQNYRLTDATLYVTFEPCVMCAGAMIHSRIGRVVFGVRNSKRGAAGSLMNVLNYPGMNHCVEITEGILVDECAALLCDFYRMPRQVLNAQKKAQSSISPGGSSGGSSGSETPGASGSVTPKSSGGSSAGSTKDTITKTLKLRIVRPYNSAEVEKIVADEKNNREKIALEKNKDKVKEACSKHLKVAAYCTTQVERNACLFCKARKLDDKFYQKLRGQFPDAVFWQEIGEIFRQLQKQAAEIYNQSLIELYYEIFIKGKGFANASSVEHYLSDVCYTRAAELFKNAAIASGLRGKVKSNFRLKELKNMKSGLPTTKSDNFPIPLVKQKGGQYTGFEISSHNDDFIIKIPFGRWQVKEEIDKYRPWEKFDFEQVRKNPKPISLLLSTQRRKGNKGWSKDEGTEAEIRKVMNGDYQTSYIEVKRGSKIGEKSAWMLNLSIDVPKVDKGVDPSIIGGIDVGVKSPLVCAINNAFSRYSISDNDLFRFNKKVFARRRILLKKNRHKRAGHGTKNKLKPITILTEKSGRFRKKLIERWACEIANFFIKNKVGTVQMEYLEGMKRKEDSYFNIRLRGFWPYAEMQNKIEFKLKQYGIKIRKVAPNNTSKTCSKCGHLNNYFSFEYRRKNKFPHFKCEKCNFKENADYNAALNISNPKLKSTKEEP

SEQ ID NO: 376 - protein, 726 aa, synthetic construct
SEVEFSHEYWMRHALTLAKRARDEREVPVGAVLVLNNRVIGEGWNRAIGLHDPTAHAEIMALRQGGLVMQNYRLSDATLYVTFEPCVMCAGAMIHSRIGRVVFGVRNSKRGAAGSLMNVLNYPGMNHCVEITEGILVDECAALLCDFYRMPRQVLNAQKKAQSSISPGGSSGGCSGSEMPGASESVTPKSSGGSSAGSTKNTITKTLKLRIVRPYNSAEVEKIVADEKNSREKIALERNKDKVKEACSEHLKVAAYCTTQVERNACLFCKARKLDDRFYQKLRGQFPDAVFWQETGEIFRQLQKQAAEIYNQSLVELYYEIFIKGKGIANASSVEHYLSDVCYTRAAELFKNAAIASGLRNKIKSNFRLKELRNMKSGLPTTKSDNFPIPLVRQKGGQYTGFEISNHNGDFIIKIPFGRWQVKKEISKHRPWEKFDFEQVRKSPKPISLLLSTQRRKRNKGWGKDEGTEAEIRKVMNGDYQTSYIEVKRGSKIGEKSAWMLNLSIDVPKIDKGVDPSIIGGIDVGVKSPLVCAINNALSRYSISDNDLFHFNKKMFARRRILLKKNRHKRAGHGARNKLKPITVLTEKSERFRKKLIERWACEIANFFIKNKVGTVQMENLESMKRKEDSYFNIRLRGFWPYAEMQNKIEFKLKQYGIKIRKVAPNNTSRTCSECGHLNNYFSFEYRKKNKFPHFKCEKCNFKENADYNAALNISNPKLKSTKEEP

SEQ ID NO: 377 - protein, 726 aa, synthetic construct
SEVEFSHEYWMRHALTLAKRARDEREVPVGAVLVLDNRVIGVGWNRAIGLHDPTAHAEIMALRQGGLVMQNYRLTDATLYVTFEPCVMCAGAMVHSRIGRVVFGVRNSKRGAAGSLMNVLNYPGMSHCVEITEGILVDECAALLCDFYRMPRQVLNAQKKAQSSISSGGSSGGSGGGETPGASESVTPKSSGGSSAGSTKNTITKTLKLRIVRPYNSAEVEKIVADEKNSREKIALEKNKDKVKEACSEHLKVATYCTTQVERNACPFCKARKLDDKFYQKLRGQFPDAVFWQELGEILRQLQKQAAEVYNQSLVELYYEIFIKGKGFANASSVEHYLSDVCYTRAAELFKNAAIASGLRGKVKSNFRLKELKNMRSGLPTTKSDNFPIPLVKQKGGQYTGFEISSHNDDFIIKIPFGRWQVKKEIDKYRPWEKFDFEQVRKSPKPISLLLSTRRRKRNKGWSKDEGTEAVIRKVMNGDYQTSYIEVKRGSKIGEKSAWMLSLSIDVPKIDKGVDPSIIGGIDVGVKSPLVCAIDSALSRYSISDNDLFHFNKKMFARRRILLKKNRHRRAGHGAKNKLKPISILTEKSKRFRKKLIERWACEIADFFIKNKVGTVQMENLESMKRKEDSYFNIRLRGFWPYAEMQNKIEFKLKQYGIEIRKVAPNNTSKTCSKCGHLNSYFNFEYRKKNKFPHFKCEKCNFRENADYNAALNISNPKLKSTKEEP

SEQ ID NO: 378 - protein, 726 aa, synthetic construct
SEGEFSHEYWMRHALTLAKRARDGREVPVGAVLVLNNRVIGEGWNRAIGLHDPTAHAEIMALRQGGLVMQNYRLIDATLYVTFEPCVMCAGAMVHSRIGRVVFGVRNSKRGAAGSLMNVLDYPGMGHRVEITEGILADECAALLCDFYCMPRQVFNAQKRAQSSISPGGSSGGSSGSETPGASESVTPKSSGGSSGGSAKNTITKTLKLRIVRPYNSAEVEKIVADEKNNREKIALEKNKDKVREACSKHLKVASYCTTQVERNACLFCKARKLDDKFYQKLRGQFPDAVFWQELGEIFRQLQKQAAEIYNQSLIELYYEIFIKGKGFANASSVEHYLSDVCYTRAAELFKNAAIASGLRGKVKSNFRLKELKNMKSGLPTTKSDNFPVPLVKQKGGQYTGFEISSHNDDFIIKIPFGRWQVRKEIDKYRPWEKFNFEQVRKSPKPISLLLSTQRRKRNKGWSKDEGTEAEIRKVMNGDYQTSYIEVKRGSKTGEKSAWMLSLSIDVPKIDKGVDPSIIGGIDVGVKSPLVCAINNAFSRYSISDNDLFRFNKKMFARRRILLKKNRHKRAGHGAKNKLKPITILTEKSERFRKKLIERWACEIADFFIKNKVGTVQMENLESMKRKEDSYFNIRLRGFWPYAEMQNKIEFKLKQYGIKIRKVAPNNTSKACSKCGHLNDYFNFEYRKKNKFPHFKCEKCNFKEDADYNAALNISNPKLKSTKEEP

SEQ ID NO: 379 - protein, 726 aa, synthetic construct
SEVEFSHEYWMRHALTLAKRARDEREVPVGAVLVLNNRVIGEGWNRAIGLHDPTAHAEIMALRQGGLVMQNYRLTDATLYVTFEPCVMCAGAMIHSRIGRVVFGVRNSKRGAAGSLMNVLNYPGMNHCVEITEGILVDECAALLCDFYRMPRQVLNAQKKAQSSISSGGSSGGSSGSETPGTSESATPKSSGGSSGGSAKNTITKTLKLRIVRPYNSAEVEKIVADEKNNREKVALEKNKDKVKEACSKHLKVAAYCTTQVERNACLFCKARRLDDKFYQKLRGQYPDAVFWQEIGEIFRQLQKQAAEIYNQSLVELYYEIFIKGKGIANASSVEHYLSDVCYTRAAELFKNAAIASGLRNKIKSNFRLKELRNMKSGLPTTKSDNFPIPLVRQKGGQYTGFEISNHNDDFIIKIPFGRWQARKEIDKYRPWEKFDFEQVRKSPKPISLLLSTQRRKRNKGWSKDEGTEAEIRKVMNGEYQTSYIEVKRGSKIGEKSAWMLNLSIDVPKIDKGVDPSIIGGIDVGVKSPLVCAINNAFSRYSISDNDLFHFNKKMFARRRILLKKNRHKRAGHGAKNKLKPISILTEKSKRFRKKLIERWACEIADFFIKNKVGTVQMENLESMKRKEDSYFNIRLRGFWPYAEMQNKIEFKLKQYGIEIRKVAPNNTSKTCSKCGHLNYYFNFEYRKKNKFPHFKCEKCNFKEDADYNAALNIGNPKLKSTKEEP

SEQ ID NO: 380 - protein, 726 aa, synthetic construct
SEVEFSHEYWMRHALTLAKRARDEREVPVGAILVLNNRVIGEGWNRAIGLHDPTAHAEIMALRQGGLVMQNYRLIDATLYVTFEPCVMCAGAMIHSRIGRVVFGVRNSKHGAAGSLVNVLNYPGMNHRVGITEGILADECAALLCDFYRMPRQVFNARKKAQSSINPGGSSGGSNGSETPGTSGSATPEGSGGSSGGSAKNTITKTLKLRIVRPYNSAEVEKIVADEKNNREKIALEKNKDKVKEACSKHLKVASYCTTQVERNACLFCKARKLDDKFYQKLRGQFPDAVFWQEIGEIFRQLQKQAAEIYNQSLVELYYEILIKGKGIANASSVEHYLSDVCYTRAAELFKNAAIASGLRNKIKSNFRLKELRNMKSGLPTTKSDNFPIPLVKQKGGQYTGFEISSHNDDFIIKIPFGRWQVKKEIDKYRPWEKFDFEQVRKSPKPISLLLSTQRRKRNKGWSKDEGTEAEIRKVMNGDYQTSYIEVKRGSKIGEKSAWMLNLSIDVPKIDKGVDPSIIGGIDVGVKSPLVCAINNALSRYSISDNDLFRFNKKMFARRRILLKKNRHKRAGHGAKNKLKPISILTEKSKRFRKKLIERWACEIADFFIKNKVGTVQMENLEGMKRKEDSYFNIRLRGFWPYAEMQNKIEFKLKQYGIEIRKVAPNNTSRTCSKCGHLNNYFNFEYRKMNKFPHFKCEKCNFKENADYNAALNISNPKLKSTKEEP

SEQ ID NO: 381 - protein, 726 aa, synthetic construct
SEVEFSHEYWMRHALTLAKRARDEREVPVGAILVLNNRVIGEGWNRAIGLHDPTAHAEIMALRQGGLVMQNHRLVDATLYVTFEPCVMCAGAMIHSRIGRVVFGVRNSKRGAAGSLTNVLNYPGMNHRVEITEGILVDECAALLCDFYRMPRQVLNAQKKARSCINSGGSSGGSSGSETPGTSESATPESSGGSSGGSAKNTITKTLKLRIVRPYNSAEVEKIVADEKDNRERIALEKNKGKVKEACSKHLKVAAYCTTQVERNACLFCKARKLDDKFYQKLRGQFPDAVFWQEIGEIFRQLQKQAAEIYNQSLIELYYEIFIKGRGFANASSVEHYLSDVCYTRAAELFKNAAIASGLRGKVKSSFRLKELKNMKSGLPTTKSDNFPIPLVKQKGGQYTGFEISSHNDDFIIKIPFGRWQVKKEIDKYRPWEKFDFEQVRKSPKPISLLLSTQRRKRNKGWSKDEGTEAEIRKVMNGDYQTSYIEVKRGSKTGEKSAWMLNLSIDVPKIDKGVDPSIIGGIDVGVKSPLVCAINNAFSRYSISDNDLFRFNKKVFARRRILLKKNRHKRAGHGTKNKLKPITILAEKSGRFRKKLIERWACEIANFFIKNKVGTVQMENLESMKRKEDSYFNIRLRGFWPYAEMQNKIEFKLKQYGIKIRKVAPNNTSKTCSKCGHLNNYFSFEYRKKNKFPHFKCEKCNFKEDADYNAALNISNPKLRSTKEEP

SEQ ID NO: 382 - protein, 726 aa, synthetic construct
SEVEFSHEYWMRRALTLAKRARDEREVPVGAVLVLNNRVIGVGWNRAVGLHDPTAHAEIMALRQGGLVMQNYRLIEATLYVTFEPCIMCAGAMIHSRIGRVVFGVRNSKRGAAGSLMNVLNYPGMNHRVEITEGILADECAALLCDYYRMPRQVFNARKKAQSSINSGGSSDGGSGSETPGTSESATPENSGGSSGGSTKNVITKALKLRIVRPYNSAEVEKIVADEKNNREKIALEKNRDKVKEACSKHLKVAAYCTTQVERNACLFCKARKLDDKFYQKLRGQFPDAVFWQELGEILRQLQKQAAEIYNQSLIELYYEIFIKGRGFANAGSVEHYLSDVCYTRAAELFKNAAIASGLRGKVKSNFRPKELKNMKSGLPTTKSDNFPIPLVKQKGGQYTGFEISSHNDDFIIKIPFGRWQVKKEIDKYRPWEKFDFEQVRKSPKPISLLLSTQRRKRNKGWSKDEGTEAEIRKVMNGDYQTSYIEVKRGSKTGEKSAWMLNLSIDVPKIDKGVDPSIIGGIDVGVKSPLVCAINNAFSRYSISDNDLFRFNKKMFARRRILLKKNRHKRAGHGAKNKLKPITILTEKSKRFRKKLIERWACEIADFFIKNKVGTVQMENLESMKRKEDSYFNIRLRGFWPYAEMQNKIEFKLKQYGIKIRKVAPNNTSRTCSECGHLNNYFSFEYRKKNKFPHFKCEKCNFKEDADYNAALNISNPKLKGTKEEL

SEQ ID NO: 383 - protein, 726 aa, synthetic construct
SEVEFSHEYWMRHALTLAKRARDEREVPVGAVLVLNNRVIGEGWNRAIGLHDPTAHAEIMALRQGGLVMQNYRLSDATLYVTFEPCVMCAGAMIHSRIGRVVFGVRNSKRGAAGSLINVLNYPGMNHCVEITEGILVDECAALLCDFYRMPRQVLSAQKKAQSSVSSGGSSGGGSGSETPGASGSVTPKSSVGSSAGSTKNTITKALKLRIVRPYNSAEVEKIVADEKNNRERIALEKNKDKVKEACSKHLKVAAYCTTQVERNACLFCKARKLDDKFYQKLRGQFPDAVFWQEIGEIFRQLQKQAAEIYNQSLIELYYEIFIKGRGFANASSVEHYLSDVCYTRAAELFKNAAIASGLRGKVKSNFRLKELRNMKSGLPTTKSDNFPIPLVRQKGGQYTGFEISNHDGDFIIKIPFGRWQVKKEINKHRPWEKFDFEQVRKSPKPISLLLSTQRRKRNKGWSKDEGTEAEIRKVMNGDYQTSYIEVKRGSKIGEKGAWMLNLSIDVPKIDKGVDPSIIGGIDVGVKSPLVCAINNALSRYSISDNDLFHFNKKMFARRRILLRKNRHKRAGHGAKNKLKPITIMTEKSKRFRKKLIERWACEIADFFIKNKVGTVQMENLESMKRKEDSYFNIRLRGFWPYAEMQSKIEFKLKQYGIVVRKVAPNNTSKTCSKCGHLNNYFNFEYRKKNKFPHFKCEKCNFKEDADYNAALNISNPKLKSTKGEP

SEQ ID NO: 384 - protein, 726 aa, synthetic construct
SEVEFSHEYWMRHALTLAKRARDEGEVPVGAVLVLNNRVIGVGWNRAIGLHDPTAHAEIMALRQGGLVMQNYRLTDATLYVTFEPCVMCAGAMVHSRIGRVVFGVRNSKRGAAGSLMNVLNFPGMSHCVEITEGILVDECAALLCDFYRMPRQVLNAQKKAQSSISSGGSSGGSGGGETPGASESVTPKNSGGSSASSTKNTITKTLKLRIVRPYNSAEVEKIVADEKNSREKIALEKNKDKVKEACSEHLKVAAYCTTQVERNACLFCKARKLDDRFYQKLRGQFPDAVFWQEIGEIFRQLQKQAAEIYNQSLVELYYEILIKGKGIANASSVEHYLSDVCYTRAAELFKNAAIASGLRNKVKSNFRLKELRNMKSGLPTTKSDNFPIPLVRQKGGQYTGFEISNHDGDFIIKIPFGRWQVKKEINKHRPWEKFDFEQVRKSPKPISLLLSTQRRKRNKGWSKDEGTEAEIRKAMNGDYQTSYIEVKRGSKIGERSAWMLSLSIDVPKIDKGVDPRIIGGIDVGVKSPLVCAINNVLSRYSISDNDLFHFNKKMFARRRILLKKNGHKRAGHGAKNKLKPITIMTEKSKRFRKKLIERWACEIADFFVKNKVGTVQMENLESMKRKEDSYFNIRLRGFWPYAEMQNKIEFKLKQYGIVVRKVAPNNTSKTCSQCGHLNNYFNFEYRKKNKFPYFKCEKCNFKENADYNAALNISSPQLKSTKGEP

SEQ ID NO: 385 - protein, 726 aa, synthetic construct
SEVEFSHEYWMRHALTLAKRARDEREVPVGAILVLNNRVIGEGWNRAIGLHDPTAHAEIMALRQGGLVMQNYRLIDATLYVTFEPCVMCAGAMIHSRIGRVVFGVRNSKHGAAGSLVNVLNYPGMNHRVEITEGILADECAALLCDFYRMPRQVFNARKKAQSSINSGGSSGGSSGSDTPGTSESATPESSGGGSSGSAKNTITKTLQLRIVRPYNSAEVEKIVADEKNNREKIALEKNKDKVREACSKHLKVASYCTTQVERNACPFCKARKLDDKFYQKLRGQFPDAVFWQELGEILRQLQKQAAEIYNQSLIELYYEIFIKGKGFANASSVEHYLSDVCYTRAAEQFKNAAIASGLRGKVKSNFRLKELKNMKSGLPTTKSDNFPIPLVRQKGGQYTGFEISSHNDDFIIKIPFGRWQVKKEIDKYRPWEKFDFEQVRKSPKPISLLLSTQRRKRNKGWSKDEGTEAEIRKVMSGDYQTSYIEVKRGSKTGEKSAWMLNLSIDVPKIDKGVDPSIIGGIDVGVRSPLVCAINNALSRYSISDNDLFHFNKKMFARRRILLKKNRRKRAGHGAKNKLKPISILTEKSERFRKKLIERWACEIADFFVKNKVGTVQMENLESMKRREDSYFNIRLRGFWPYAKMLNKIEFKLKQYGIKIRKVAPNNTSKTCSKCGHLNNYFNFEYRKKNKFPHFKCEKCNFKENADYNAALNISNPKLKSTKGEP

SEQ ID NO: 386 - protein, 726 aa, synthetic construct
SEVEFSHEYWMRHALTLAKRARDEREVPVGAVLVLNNRVIGEGWNRAIGLHDPTAHAEIMALRQGGLVMQNYRLTDATLYVTFEPCVMCAGAMIHGRISRVVFGVRNGKRGAAGSLMNVLNYPGMNHCVEITEGILVDECAALLCDFYHMPRQVLNAQKKAQSGISSGGSSGGSSGSETPGASVSVTPKSSGGSSADSTKDTITKTLKLRIVRPYNSAEVEKVVADEKNNREKIAIEKNKDMVKEACSKHLKVASYCTTQVERNACLFCKARKLDDKFYQKLRGQFPDAVFWQELGGIFRQLQKQAAEIYNQSLIELYYEIFIKGKGITNASRVEHYLSDVCYTRAAELFKNAAIASGLRGKVKSNFRLKELKNMKSGLPTTKSDNFPIPLVKQKGGQYTGFEISSHNDDFIIKIPFGRWQVKKEIGKYRPWEKFDFEQVRKSPKPISLLLSTRRRKKNKGWSKDEGTEAEIRKVMNGDYQTSYIEVKRGSKIGEKSAWMLNLSIDVPKIDKGVDPSIVGGIDVGVKSPLVCAINNAFSRYSIGDNDLFHYNKKMFARRRILLKKNRHKRAGHGAKNKLKPISILTEKSKRFRKKLIERWACEIANFFIKNKVGTVQMENLESMKRKEDSYFNIRLRGFWPYAEMQNKIEFKLKQYGIKIRKVAPNNTSKTCSKCGHLNNYFSFEYRKKNKFPHFKCEKCNFKEDADYNAALNISNPKLKSTKEEP

SEQ ID NO: 387 - protein, 726 aa, synthetic construct
SEVEFSHEYWMRHALTLAKRARDEREVPVGAILVLNNRVIGEGWNRAIGLHDPTAHAEITALRQGGLVMQNYRLIDATLYVTFEPCVMCAGAMIHSRIGRVVFGVRNSKHGAAGSLVNVLNYPGMNHRVEITEGILADECAALLCDFYRMPRQVFNARKKAQSSIDPGGSSGGSGGSETPGTSESTTPEGSGSSSGGSAKNTITKTLKLRIVRPYNSAEVEKIVANEKNNREKIALEKNKDKVKEACSKHLKVASYCTTQVERNACPFCKARKLDDKFYQKLRGQFPDAVFWQELGGIFRQLQKQAAEIYNQSLIELYYEIFIKGKGITNASRVEHYLSDVCYTRAAELFKNAAIASGLRGKVKSNFRLRELKNMKSGLPTTKSDNFPIPLVKQKGGQYTGFEISNHNSDFIIKIPFGRWQVKKEINKYRPWEKFDFEQVRKSPKPISLLLSTQRRKRNKGWSKDEGTEAEIRKVMNGDYQTSYIEVKRGSKIGEKSAWMLNLSIDVPKIDKGVDPSIIGGIDVGVKSPLVCAINNAFSRYSISDNDLFRFNKKMFARRRILLGKNRHKRAGHGVKNKLKPITILTEKSGRFRKKLIERWACEIADFFVKNKVGTVQMENLESMKRKEDSYFNIRLRGFWPYAEMQNKIEFKLKQYGIEVRKVAPNNTSKTCSKCGHLNNYFNFEYRKKNKFPHFKCEKCNFKENADYNAALNISNPKLKSTKEEP

SEQ ID NO: 388 - protein, 726 aa, synthetic construct
SEVEFSHEYWMRHALTLARRARDEREVPVGAILVLNNRVIGEGWNRAIGLHDPTAHAEIMALRQGGLVMQNYRLIDATLYVTFEPCVMCAGAMVHSRIGRVVFGVRNSKRGAAGSLMNVLDYPGMGHRVEITEGILADECAALLCDFYCMPRQVFNAQKRAQSSINSGGASGGSSGSETPGASGSVTPKGSVGSSAGSTKNTITKTLKLRIVRPYNSAEVEKIVADEKNNREKIALEENKDKVKEACSKHLKVAAYCTTQVERNACLFCKARKLDDKFYQKLRGQFPDAVFWQELGGIFRQLQKQAAEIYNQSLIELYYEIFIKGKGITNASRVEHYLSDVCYTRAAELFRNAAIASGLRSKVRSNFRLKELKNMKSGLPTTKSDNFPIPLVKQKGGQYTGFEISSHNDDFIIKIPFGRWQVKKEIDRYRPWEKFDFEQVRKSPKPISLLLSTQRRKRNKGWSKDEGTEAEIRKVMNGDYQTSYIEVKRGSKIGEKSAWMLNLSIDVPKIGKGVDPSIIGGIDVGVKSPLVCAINNAFSRYSISDNDLFRFNKKMFARRRILLKKNRHRRAGHGAKNKLKPITILTEKSKRFRKKLIERWACEIADFFIKNKVGTVQMENLESMKRKEDSYFNIRLRGFWPYAEMQNKIEFKLKQYGVKVRKVAPNNTSRTCSRCGHLNNYFSFEYRKKNKFPHFKCEKCNFKEDADYNAALNISNPKLKGTKEEL

SEQ ID NO: 389 - protein, 726 aa, synthetic construct
SEVEYSHEYWMRYALTLAKRARDEREVPVGAVLVLNNRVIGEGWNRAIGLHDPTAHAEIMALRQGGLVMQNYRLIDATLYVTFEPCVMCAGAMIHSRIGRVVFGVRNNKHGAAGSLVNVLNYPGMNHRVEITEGILADECAALLCDFYRMPRQVFNARKKAQSSINPGGSSGSSRGSETPGTSESAAPGSSGGNSGGSAKNTITKTLKLRIVRPYNSAEVEKIVADEKNNREKIALEKNKDKVKEACSEHLKVAAYCTTQVERNACLFCKARKLDDKFYQKLRGQFPDAVFWQEIGEIFRQLQKQAAEIYNQSLIELYYEIFIKGKGFANASSVEHYLSDVCYTRAAELFKNAAIASGLRGKVKSNFRLKELKNMRSGLPTTKSDNFPIPLVKQKGGQYAGFEISSHNDDFIIKIPFGRWQVKKEIDKYRPWEKFDFEQVRKSPKPISLLLSTRRRKRNKGWSKDEGTEAEIRKVMNGDYQTSYVEVKRGSKIGEKSAWMLNLSIDVPKIDKGVDPSIIGGIDVGVKSPLVCAINNAFGRYSISDNDLFHFNKKMFAMRRILLKKNRHKRAGHGAKNKLKPITILTEKSKRFRKKLIERWACEIADFFIKNKVGTVQMENLESMKRKEDSYFNIRLRGFWPYAEMQGKIEFKLKQYGIEIRKVAPNNTSKTCSRCGHLNNYFNFEYRRKNKFPHFKCEKCNFKENADYNAALNISNPKLKSTKEEP

SEQ ID NO: 390 - protein, 726 aa, synthetic construct
SEVEFSHEYWMRHALTLAKRARDEREVPVGAVLVLNNRVIGEGWNRAIGLHDPTAHAEIMALRQGGLVMQNYRLIDATLYVTFEPCAMCAGAVVHSRVGRVVFGVRNSKRGAAGSLMNVLNYPGMDHRVEITGGILADECAALLCDFYRMPRRVFNAQKKAQSSINSGGSSGGSSGSVTPGTSESATPESSGGSFGGSAKNTITKTLQLRIVRPYNSAEVEKIVADEKNSREKIALEKNKDKVKEACGKHLKVASYCTTQVERNACLFCKARKLDDKFYQKLRGQFPDAVFWQELGEIFRQLQKQAAEIYNQSLIELYYEIFIKGKGLANASSVEHYLSDVCYTRAAELFKNAAIASGLRGKVKSNFKLKELKSMKSGLPSTKSDNFPIPLVKQKGGRYTGFEISSHNDDFIIKIPFGRWQVKEEIDKYRPWEKFDFEQVRKNPKPISLLLSTQRRKGNKGWSKDEGTEAEIRKVMNGDYQTSYIEVKRGSKIGEKSAWMLNLSIDVPKIDKGVDPSIIGGIDVGVKSPLVCAINNAFSRYSISDNDLFRFNKKVFARRRILLKKNRHKRAGHGTKNKLKPITILTEKSGRFRRKLIERWACEIANFFIKNKVGTVQMENLESMKRKEDSYFNIRLRGFWPYAEMQNKIEFKLKQYGIKIRKVAPNNTSKTCSRCGHLNNYFSFEYRKKNKFPHFKCEKCNFKEDADYNAALNISNPKLKSTKEEP

SEQ ID NO: 391 - protein, 726 aa, synthetic construct
SEVEFSHEYWMRRALTLAKRARDEREVPVGAVLVLNNRVIGVGWNRAVGLHDPTAHAEIMALRQGGLVMQNYRLIEATLYVTFEPCIMCAGAMIHSRIGRVVFGVRNSKRGAAGSLMNVLNYPGMNHRVEITEGILADECAALLCDFYRMPRQVFNARKKAQSSINSGGSSGGSSGSETPGTSESATPESSGGSSGGSAKNTITKALKLRIVRPYNSAEVEKIVADEKNNRERIALEKNKDKVKEACSKHLKVAAYCTTQVERNACLFCKARKLDDKFYQKLRGQFPDAVFWQEIGEIFRQLQKQAAEIYNQSLIELYYEIFIKGKGFANASSVEHYLSGVCYTRAAELFKNAAIASGLRGKVKSNFRLKELKNMRSGLPTTKSDNFPIPLVKQKGGQYTGFEISSHNDDFIIKIPFGRWQVKKEIDKYRPWEKFDFEQVRKSPKPISLLLSTRRRKRNKGWSKDEGTEAEIRKVMNGNYQTSYIEVKRGSKTGEKSTWMLNLSIDVPKIDKGVDPSIIGGIDVGVKSPLVCAINNAFSRYSISDNDLFRFNKKMFARRRILLKKNRHKRAGHGAKNKLKPISILTEKSKRFRKKLIERWACEIADFFIKNKVGTVQMENLESMKRKEDSYFNIRLRGFWPYAEMQNKIEFKLRQYGIEIRKVAPNNTSKTCSKCGHLNNYFNFEYRRKNKFPHFKCEKCNFKEDADYNAALNISNPKLKSTKEEP

SEQ ID NO: 392 - protein, 726 aa, synthetic construct
SEVEFSHEYWMRHALTLAKRARDEREVPVGAILVLNNRVIGEGWNRAIGLHDPTAHAEIMALRQGGLVMQNYRLIDATLYVTFEPCVMCAGAMIHSRIGRVVFGVRNSKHGAAGSLVNVLNYPGMNHRVEITEGILADECAALLCDFYRMPRQVFSARKKAQSSINPGGSSGGSSGSGTPGTSESATPESSGGSSAGSTKNTITKTLKLRIVRPYNSAEVEKIVADEKNSREKIALERNKDKVKEACSEHLKVAAYCTTQVERNACLFCKARKLDDRFYQKLRGQFPDAVFWQETGEIFRQLQRQAAEIYNQSLIELYYEIFIKGKGFANASSVEHYLSDVCYTRAAELFKNAAIASGLRGKVKSNFRLKELKNMKSGLPTTKSDNFPIPLVKQKGGQYTGFEISSHNDDFIIKIPFGRWQVKKEINKYRPWEKFDFEQVRKSPKPISLLLSTQRRKRNKGWSKDEGTEAEIRKVMNGDYQTSYIEVKRGSKIGEKSAWMLNLSIDVPKIDKGVDPSIIGGIDVGVKSPLVCAINNAFGRYSISDNDLFHFNKKMFARRRILLKKNRHKRAGHGAKNKLKPITILTEKSKRFRKKLIERWACEIADFFIKNKVGTVQMENLESMKRKEDSYFNIRLRGFWPYAEMQDKIEFKLKQYGIEIRKVAPNNTSKTCSRCGHLNNYFDFEYRRKNKFPHFKCEKCNFKENADYNAALNISNPKLKSTKEEP

SEQ ID NO: 393 - protein, 726 aa, synthetic construct
SEVEFSHEYWMRHALTLAKRARDEREVPVGAVLVLNNRVIGEGWNRAIGLHDPTAHAEIMALRQGGLVMQNYRLTDATLYVTFEPCVMCAGAMIHSRIGRVVFGVRNSKRGAAGSLMNVLNYPGMNHRVEITEGILADECAALLCDYYRMPRQVFNARKKAQSSINSGGSSDGGSGSETPGTSESATPESSGGSSGGSAKNTITKTLKLRIVRPYNSAEVEKIVADEKSNREKIALEKNKDKVKEACSEHLKVAAYCTTQVERSACLFCKARKLDDKFYQKLRGQFPDAVFWQELGEILRQLQKQAAEIYNQSLIELYYEIFIKGRGFANASSVEHYLSDVCYTRAAELFKNAAIASGLRGKVKSNFRLKELKNMKSGLPTTKSDNFPIPLVKQKGGQYTGFEISSHNSDFIIKIPFGRWQEKEEIDKYRPWEKFDFEQVRKSPKPISLLLSTQRRKKNKGWSKDEGTEAEIRRVMNGDYQTSYIEVKRGSKIGEKSAWMLNLSIDVPKIDKGVDPSIIGGIDVGVKSPLVCAINNAFSRYSISDNDLFHFNKKMFARRRILLKKNRHRRAGHGAKNKLKPITILTEKSVRFRKKLIERWACEIADFFIKNKVGTVQMENLESMKRKEDSYFNIRLRGFWPYAEMQNKIEFKLKQYGIEIRRVAPNNTSRTCSKCGHLNNYFNFEYRRKNKFPHFKCEKCNFKEDADYNAALNISNPKLKSTKEEP

SEQ ID NO: 394 - protein, 726 aa, synthetic construct
SEVEFSHEYWMRRALTLAKRARDEREVPVGAVLVLNNRVIGVGWNRAVGLHDPTAHAEIMALRQGGLVMQNYRLVEATLYVTFEPCIMCAGAMIHSRIGRVVFGVRNSKRGAAGSLMNVLNYPGMNHRVEITEGILADECAALLCDYYLMPRQVFNARKKAQSSINSGGSSDGGSGSETPGTSESATPESSGGSSGGSAKNTITKTLKLRIVRPYNSAEVEKIVADEKDNREKIALEKNKDKVKEACSEHLRVAAYCTTQVERSACLFCKARKLDDKFYQKLRGQFPDAVFWQEIGEIFRQLQKQAAEIYNQSLIELYYEIFIKGKGFANASSVEHYLSDVCYTRAAELFKNAAIASGLRGKVKSNFRLKELKNMKSGLPTTKSDNFPIPLVKQKGGQYTGFEISSHNDDFIIKIPFGRWQVKKEIDKYRPWEKFDFEQVRKSPKPISLLLSTQRRKRNKGWSKDEGTEAEIRKVMNGDYQTSYIEVKRGRKIGEKSAWMLSLSIDVPKIDKGVDPRIIGGIDVGVKSPLVCAINNVLSRYSISDNDLFHFNKKMFARRRILLKKNGHKRAGHGAKNKLKPITIMTEKSRRFRKKLIERWACEIADFFIKNKVGTVQMENLESMKRKEDSYFNIRLRGFWPYAEMQNKIEFKLKQYGIVVRKVAPNNTSKTCSQCGHLNNYFNFEYRKKNKFPYFKCEKCNFKENADYNAALNISNPKLKSTKEEP

SEQ ID NO: 395 - protein, 726 aa, synthetic construct
SEVEFSHEYWMRHALTLAKRARDEREVPVGAVLVLNNRVIGEGWNRAIGLHDPTAHAEIMALRQGGLVMQNYRLVDATLYVTFEPCVLCAGAMVHSRIGRVVFGVRNSKRGAAGSLMNVLNYPGMNHRVEITEGILADECAALLCDFYRMPRQVFNARKKARSNINSSGPSGGSSDSETPGASESITPRSSGGSSGGSAKNTITKTLKLRIVRPYNSAEVEKIVADEKNNREKIALEKNKDKVKEACGKHLKVASYCTTQVERNACLFCKARKLDDKFYQKLRGQFPDAVFWQELGEIFRQLQKQAAEIYNQSLIELYYEIFIKGKGLANASSVEHYLSDVCYTRAAELFKNAAIASGLRNKVKSNFRLKELRSMKSGLPTTKSDNFPIPLVRQKGGQYTGFEISSHNDDFIIKIPFGRWQVKKEIDRYRPWEKFDFEQVRKSPKPISLLLSTQRRKRNKGWSKDEGTEAEIRKVMNGDYQTSYIEVKRGSKIGEKSAWVLNLSIDVPKIDKGVDPSIIGGIDVGVKSPLVCAINNAFSRYSISDNDLFHFNKKMFARRRILLKKNRHKRAGHGAKNKLKPISILTEKSKRFRKKLIERWACEIADFFIKNKVGIVQMENLESMKRKEDSYFNIRLRGFWPYAEMQNKIEFKLKQHGIEIRKVAPNNTSKTCSKCGHLNNYFNFEYRKMNKFPHFKCEKCNFKENADYNAALNISNPKLKSTKEEP

SEQ ID NO: 396 - protein, 726 aa, synthetic construct
SEVEFSHEYWMRHALTLAKRARDEREVPVGAVLVLNNRVIGEGWNRAIGLHDPTAHAEIMALRQGGLVMQNYRLIDATLYVTFEPCVMCAGAMIHSRIGRVVFGVRNNKHGAAGSLMNVLNYPGMNHRVEITEGILADECAALLCDFYRMPRQVFNARKKAQSSINPGGSSGGSGGSETPGTSESATPENSGGSSGSSAKNTITKTLKLRIVRPYNSAEVEKIVADEKNNREKIALEKNKDKVKEACSKHLKVAAYCTTQVERNACQFCRARKLDDKFYQKLRGQFPDAVFWQEIGEIFRQLQKQAAEIYNQSLIELYYEIFIKGRGFANASSVEHYLSDVCYTRAAELFKNAAIASGLRGKVKSNFRLKELKNMKSGLPTTKSDNFPIPLVKQKGGQYTGFEISSHNDDFIIKIPFGRWQVKKEIDKYRPWEKFDFEQVRKSPKPISLLLSTQRRKRNKGWSKDEGTEAEIRKVMNGDYQTSYIEVKRGSKTGEKSAWMLSLSIDVPKIDKGVDPSIIGGIDVGVKSPLVCAINNAFNRYSISDNNLFHFNKKMFARRRILLKKNRHKRAGHGAKNKLRPISILTEKSERFRKKLIERWACEIADFFIRNKVGTVQMENLEGMKRKEDSYFNIRLRGFWPYAEMQNKIEFKLKQYGIEVRKVAPNNTSKTCSKCGHLNNYFNFEFRKKNKFPHFKCEKCNFKENADYNAALNISNPKLKSAKEEP

SEQ ID NO: 397 - protein, 726 aa, synthetic construct
SEVEFSHEYWMRHALTLAKRARDEREVPVGAVLVLNNRVIGEGWNRAIGLHDPTAHAEIMALHQGGLVMQNYRLIDATLYVTFEPCVMCAGAMIHSRIGRVVFGARNSKRGAAGSLMNVLSYPGMNHRVEITEGILADECAALLCDFYRMPRRVFNAQKKAQSSINSGGSSGGGSGSDTPSTSESTTPESSGGSSGGPAKNTITKTLKLRIVRPYNSAEVEKIVADEKNNREKTALEKNKDKVKEACSKHLKVATYCTTQVERNACLFCKARKLDDKFYQKLRGQFPDAVFWQEIGEIFRQLQKQAAEIYNQSLIELYYEIFIEGKGFANASSVEHYLSDVCYTRAAELFKNAAIASGLRGKVKGNFRLKELKSMKSGLPTTKSDNFPIPLVKQKGGQYTGFEISSHNDDFIIKIPFGRWQVKKEIDKYRPWEKFDFEQVRKSPKPISLLLSTQRRKRNRGWSKDEGTEAEIRRVMNGDYQTSYIEVKRGSKIGEKSAWMLNLSIDVPKIDKGVDPSIIGGIDVGVKSPLVCAINNAYSRYSISDNDLFHFNKKMFARRRILLKKNRHKRAGHGARNKLKPITILTEKSERFRKKLIEKWACEIADFFIKNKVGTVQMENLESMKRREDSYFNIRLRGFWPYAKMLDKIEFKLKQYGIKIRKVAPNNTSKTCSKCGHLNNYFNFEYRKKNKFPHFKCEKCNFKENADYNAALNISNPKLKSTKGEP

SEQ ID NO: 398 - protein, 726 aa, synthetic construct
SEVEFSHEYWMRHALSLAKRARDEREVPVGAVLVLNNRIIGEGWNRAIGQHDPTAHAEIMALRQGGLVMQNNRLTDATLYVTFEPCVMCAGAMVHSRIGRVVFGVRNSKRGAAGSLMNVLNYPGMNHRVEITEGILVDECAALLCDFYRMPRQVFNAQKKAQSTINSGGSSGGSSGSETPGTSESATPESSGGGSSGSAKNTITKTLQLRIVRPYNSAEVEKIVADEKNNREKIALEKNKDKVKEACSKHLKVASYCTTQVERNACPFCKARKLDDKFYQKLRGQFPDAVFWQELGEILRQLQKQAAEIYNQSLIELYYEIFIKGRGFANASSVEHYLSDVCYTRAAELFRNAAIASGLRGKVKSNFRLKELKNMKSGLPTTKSDNFPIPLVKQKGGQYTGFEISSHDDDFIIKIPFGRWQVKKEIDKYRPWEKFDFEQVRKSPKPISLLLSTQRRKRNKGWSKDEGTEAEIRKVMNGDYQTSYIEVKRGSKTGEKSAWMLNLSIDVPKIDKGVDPSIIGGIDVGVKSPLVCAINNAFSRYSISDNDLFHFNKKMFARRRILLKKNGHKRAGHGAKNKLKPITIMTEKSKRFRKKLIERWACEIADFFIKNKVGTVQMENLESMKRKEDSYFNIRLRGFWPYAEMQNKIEFKLKQYGIVVRKVAPNNTSKTCSQCGHLNNYFNFEYRKKNKFPYFKCEKCNFKENADYNAALNISNPQLKSTRGEP

SEQ ID NO: 399 - protein, 726 aa, synthetic construct
SEVEFSHEYWMRHALALAKRARDEREVPVGAVLVLNNRVIGEGWNRAIGLHDPTAHAEIMALRQGGLVMQNYRLTDATLYVTFEPCVMCAGAMIHSRIGRVVFGVRNSKRGAAGSLMNVLNYPGMDHCVEITEGILVDECAALLCDFYRMPRQVLNAQKKAQSSISSGGSSGGSSGSVTPGASGSVTPKSSGGSSAGSTKDTITKTLKLRIVRPYNSAEVEKIVADEKNNREKIALEKNKDKVKEACSKHLKVASYCTTQVERNACPFCKARKLDDKFYQKLRGQFPDAVFWQELGEILRQLQKQAAEIYNQSLIELYYEIFIKGRGFANASSVEHYLSDVCYTRAAELFKNAAIASGLRGKVKSNFRLKELKNMKSGLPTTKSDNFPIPLVKQKGGQYTGFEISSHNDDFIIKIPFGRWQVKKEIDKYRPWEKFDFEQVRKSPKPISLLLSTQRRKRNKGWSKDEGTEAEVRKVMNGDYRTSYIEVKRGSKTGEKSAWMLNLSIDVPKIDKGVDPSIIGGIDVGVKSPLVCAINNAFSRYSISDNDLFRFNKKMFARRRILLKKNRHQRAGHGAKNKLKPITILTEKSGRFRKKLIERWACEIADFFIKNKVGTVQMENLESMKRKEDSYFNIRLRGFWPYAEMQNKIEFKLKQYGIKIRKVAPNNTSKTCSKCGHLNNYFNFEYRKKNKFPHFKCEKCNFKENADYNAALNICNPKLKSTKEEP

SEQ ID NO: 400 - protein, 726 aa, synthetic construct
SEVEFSHEYWMRHALTLAKRARDEREVPVGAVLVLNNRVIGEGWNRAIGLHDPTAHAEIMALRQGGLAMQNYRLVDATLYVTFEPCVLCAGAMVHSRIGRVVFGVRNSKRGAAGSLMNVLNHPGMNHRVEITGGILADECAALLCDFYRMPRQVFNAQKKARSNINSGGSSGGSSGSETLGTSESATPESSGGSSGGSAKNTITKTLKLRIVRPYNSAEVEKIVADEKNNREKIALEKNKDKVKEACSEHLKVAAYCTTQVERNACLFCKARKLDDKFYQKLRGQFPDAVFWQEIGEIFRQLQRQAAEIYNQSLIELYYEIFIKGKGFANASSVEHYLSDVCYARAAELFKNAAIASGLRGKVKSNFRLKELKNMKSGLPTTKSDNFPIPLVKQKGGQYTGFEISSHNDDFIIKIPFGRWRVKKEIDKYRPWEKFDFEQVRKSPKPISLLLSTQRRKRSKGWSKDEGTEAEIRKVMNGDYQTSYIEVKRGSKIGEKSAWMLSLSIDVPKIDKGVDPSIIGGIDVGVKSPLVCAINNAFCRYSISDNDLFHFNKKMFARRRILLKKSRHKRAGHGAKNKLKPISILTEKSKRFRKKLIERWACEIADFFIKNKVGTVQMENLESMKRKEDSYFNIRLRGFWPYAEMQNKIEFKLKQYGIKIRKVAPNNTSKTCSKCGHLNNYFSFEYRKKNKFPHFKCEKCNFKEDADYNAALNISNPKLKSTKEEP

SEQ ID NO: 401 - protein, 726 aa, synthetic construct
SEVEFSHEYWMRHALTLAKRARDEREVPVGAVLVLNNRVIGEGWNRAIGLHDPTAHAEIMALRQGGLVLQNYRLVDATLYVTFEPCVLCAGAMVHSRIGRVVFGARNSKRGAAGSLMNILNYPGMNHRVEITEGILADECAALLCDFYRMPRQVFNAQKKAQSSINSGGSSGGSSGSETPSTSESATPESSGGSSGGSAKNTITKTLQLRIVRPYNSAEVEKIVTDEKNNREKIALEKNKDKVKEACSKHLKMASYCTTQVERNACLFCKARKLDDKFYQKLRGQFPDAVFWQELGGIFRQLQKQAAEIYNQSLIELYYEILIKGKGIANASSVEHYLSDVCYTRAAELFKNAAIASGLRNKIKSNFRLKELRNMRSGLPTTKSDNFPIPLVKQKGGQYTGFEISSHNDDFIIKIPFGRWQVKKEIDKYRPWEKFNFEQVRKSPKPISLLLSTQRRKRNKGWSKDEGTEAEIRKVMNGDYQTSYIEVKRGSKTGEKSAWMLNLSIDVPKIDKGVDPSIIGGIDVGVKSPLVCAINNALSRYSISDNDLFRFNKKMFARRRILLKKNRHKRAGHGAKNKLKPISILTEKSKRFRKKLIERWACEIADFFIKNKVGTVQMENLESMKRKEDSYFNIRLRGFWPYAEMQNKIEFKLKQYGIEIRKVAPNNTSKTCSRCGHLNNYFNFEYRKKNKFPHFKCEKCNFKENADYNAALNISNPKLKSTKEKP

SEQ ID NO: 402 - protein, 726 aa, synthetic construct
SEVEFSHEYWMRHALTLAKRARDEREVPVGAILVLNNRVIGEGWNRAIGLHDPTAHAEIMALRQGGLVMQNYRLIDATLYVTFEPCVMCAGAMIHSRIGRVVFGVRNSKHGAAGSLVNVLNYPGMNHRVEITEGILADECAALLCDFYRMPRQVFGARRKAQSSINPGGSSGGSSGSETPGTGKSPTPESPGGSSGGSAKNTITKTLKLRIVRPYNSAEVEKIVADEKNNREKIALEKNKDKVKEACSKHLKVAAYCTTQVERNACLFCKARKLDDKFYQKLRGQFPDAVFWQEIGEIFRQLQKQAAEIYNQSLIELYYEIFIKGRGFANASSVEHYLSDVCYTRAAELFKNAAIASGLRGKVKSNFRLKELKNMKSGLPTTKSDNFPIPLVKQKGGQYTGFEISSHNDDFIIKIPFGRWQAKKEIDKYRPWEKFDFEQVRKSPKPISLLLSTQRRKRNKGWSKDEGTEAEIRKVMNGDYQTSYIEVKRGSKTGEKSAWMLSLSIDVPKIDKGVDPSIIGGIDVGVKSPLVCAINNAFSRYSISDNDLFRFNKKMFARRRILLKKNRHKRAGHGAKNKLKPITILTEKSRRFRKKLIERWACEIADFFIKNKVGTVQMENLESMKRKEDSYFNIRLRGFWPYAEMQNKIEFKLKQYGIEIRKVAPNNTSKTCSKCGHLNNYFNFEYRKMNKFPHFKCEKCSFKEDADYNAALNISNPRLKSTKEEP

SEQ ID NO: 403 - protein, 726 aa, synthetic construct
SEVEFSHEYWMRRALTLAKRARDEREVPVGAVLVLNNRVIGVGWNRAVGLHDPTAHAEIMALRQGGLVMQNYRLVEATLYVTFEPCIMCAGAMIHSRIGRVVFGVRNSKRGAAGSLMNVLNYPGMNHRVEITEGILADECAALLCDYYRMPRQVFNARKKAQSSINSGGSSDGGSGSETPGTSESATPESSGGSSGGSAKNTITKTLKLRIVRPYNSAEVEKIVADEKNSREKIAMEKNKDKVKEACSKHLKVASYCTTQVERNACLFCKARKLDDKFYQKLRGQFPDAVFWQELGGIFRQLQKQAAEIYNQSLIELYYEIFIKGKGITNASRVEHYLSDVCYTRAAELFKNAAIASGLRGKVKSNFRLKELKNMKSGLPTTKSDNFPIPLVKQKGGQYTGFEISSHNDDFIIKIPFGRWQVKKEIDKYRPWEKFDFEQVRKSPKPISLLLSTQRRKRNKGWSKDEGTEAEIRKVMNGDYQTSYIEVKRGSKTGEKSAWMLNLSIDVPKIDKGVDPSTIGGIDVGVKSPLVCAINNAFSRYSISDNDLYRFNKKMFARRRILLKKNRHKRAGHGAKNKLKPISILTEKSERFRKKLIERWACEIADFFIKNKVGTVQMENLESMKRREDSYFNTRLRGFWPYAEMQNKIEFKLKQYGIVVRKVAPNNTSKTCSKCGHLNNYFNFEYRKRNKFPHFKCEKCNFKEDADYNAALNISNPMLKSTKGEP

SEQ ID NO: 404 - protein, 726 aa, synthetic construct
SEVEFSHEYWMRHALTLAKRARDEREVPVGAILVLNNRVIGVGWNRAIGLHDPTAHAEIMALRQGGLVTQNYRLINATLYVTFEPCVMCAGAMIHSRIGRVVFGVRNSKHGAAGSLVNVLNYPGMNHRVEITEGILADECAALLCDFYRMPRQVFNARKKARSSINSGGSSGGSSGSETPGASGSATPKSSGGSSGGSAKNTITKTLKLRIVRPYNSAEVEKIVADEKNNREKIALEKNKDKVKEACSKHLKVAAYCTTQVERNACLFCRARKLDDKFYQKLRGQFPDAVFWQEIGEILRQLQKQAAEIYNQSLIELYYEIFIKGKGFANASSVEHYLSDVCYTRAAELFKNAAIASGLRGKVKSNFRLKELKNMKSGLPTTKSDNFPIPLVKQKGGQYTGFEISNHNDDFIIKIPFGRWQVKKEINKYRPWEKFDFEQVRKSPKPISLLLSTQRRKRNKGWSRDEGTEAEIRRVMNGDYQTSYIEVKRGSKIGEKSAWMLNLSIDVPKIDKGVDPSIIGGIDVGVKSPLVCAINNAFSRYSISDNDLFHFNKKMFARRRILLKKTRHKRAGHGAKNKLKPISILTEKSERFRKKLIERWACEIADFFIKNKVGTVQMENLESMKRREDSYFNIRLRGFWPYAKMQNKIEFKLKQYGIEIRKVAPNNTSKTCSKCGHLNNYFNFEYRKKNKFPHFKCEKCNFKENADYNAALNISNPKLKSTKEEP

SEQ ID NO: 405 - protein, 726 aa, synthetic construct
SEVEFSHEYWMRHALTLAKRARDEREVPVGAILVLNNRVIGEGWNRAIGLHDPTAHAEIMALRQGGLVMQNYRLIDATLYVTFEPCVMCAGAMVHSRIGRVVFGVRNSKRGAAGSLMNVLDYPGMGHRVEITEGILADECAALLCDFYCMPRQVFNAQKRAQSSINSGGSSGGSSGSETPGASGSVTPKSSVGSSAGSTKNTITKTLKLRIVRPYNSAEVEKIVADEKNNREKIALEKNKGKVKEACSKHLKVASYCTTQVERNACPFCKARKLDDKFYQKLRGQFPDAVFWQELGGILRQLQKQAAEIYNQSLIELYYEIFIKGRGFANASSVEHYLSDVCYTRAAGLFKNAAIASGLRGKVKSNFRLKELKNTKSGLPTTKSDNFPIPLVKQKGGQYTGFEISSHNDDFIIKIPFGRWQVKEEIDKYRPWEKFDFEQVRKNPKPISLLLSTQRRKRNKGWSKDEGTEAEIRRVMNGDYQTSYIEVKRGSKIGEKSTWMLNLSIDVPKIDKGVDPSIIGGIDVGVKSPLVCAINNAFSRYSISDNDLFRFNKKVFARRRILLKKNRHKRAGHGTKNKLKPITILAEKSGRFRKKLIERWACEIANFFIKNKVGTVQMENLESMKRKEDSYFNIRLRGFWPYAEMQNKIEFKLKQYGIKIRKVAPNNTSKTCSKCGHLNNYFNFEYRKKNKFPHFKCEKCNFKENADYNAALNISNPKLKSTKEEP

SEQ ID NO: 406 - protein, 726 aa, synthetic construct
SEVEFSHEYWMRHALTLAKRARDGREVPVGAVLVLNNRVIGEGWNRTTGLHDPTAHAEIMALRQGGLVMQNHRLVDATLYVTFEPCVMCAGAMIHSRIGRVVFGVRNSKRGAAGSLTNVLDYPGMNHRVEITEGILVDECAALLCDFYRMPRQVFNARKKAQSTINSGGSSGGSSGSETPGASESVTPKSSGGSSGGSAKNTITKTLKLRIVRPYNSAEVEKIVADEKNNREKIALEKNKGKVKEACSKHLEVAAYCTTQVERNACLFCKARKLDDKFYQKLRGQFPDAVFWQELGEIFRQLQKQAAEIYNQSLIELYYEIFIKGKGFANASSVEHYLSDVCYTRAAELFKNAAIASGLRGKVKSNFRLKELKNMKSGLPTTKSDNFPIPLVKQKGGKYAGFEISSHNDDFIIKIPFGRWQVKKEIDKYRPWEKFDFEQVRKSPKPISLLLSTQRRKRNKGWSKDEGTEAEIRKVMSGDYQTSYIEVKRGSKIGEKSAWMLNLSIDVPKIDKGVDPSIIGGIDVGVKSPLVCAINNAFSRYSISDNDLFHFNKKMFARRRILLKKNRHKRAGHGAKNKLKPISILTEKSKRFRKKLIERWACEIADFFVKNKVGTVQMENLESMKRKEDSYFNIRLRGFWPYAEMQNKIEFKLKQYGIEIRKVAPNNTSKTCSKCGHLNNYFNFEYRKKNKFPHFKCEKCNFKENADYNAALNISNPRLKSTKEEP

SEQ ID NO: 407 - protein, 726 aa, synthetic construct
SEVEFSHEYWMRHALTLAKRARDEREVPVGAVLVLNNRVIGVGWNRAIGLHDPTAHAEIMALRQGGLVTQNYRLVDATLYVTFEPCVMCAGAMIHSRIGRVVFGVRNGKRGAAGSLMNVLNYPGMNHRVEITEGILADECAALLCDFYRMPRQVFNAQKKAQSNINSGSSSGGSSGSETPGTSESATPVSSSGSSGGSAKNTITKTLKLRIVRPYNSAEVEKIVADEKNNRERVALEKNKDKVKEACSKHLKVAAYCTTQVERNACLFCKARKLDDKFYQKLRGQFPDAVFWQELGEILRQLQKQAAEIYNQSLIELYYEIFIKGKGFANASSVEHYLSDVCYTRAAELFKNAAIASGLRGKVKSNFRLKELKNMKSGLPTTKSDNFPIPLVKQKGGQYTGFEISSHNDDFIIKIPFGRWQVKKEVDKYRPWEKFDFEQVRKSPKPISLLLSTQRRKKNKGWSKDEGTEAEIRRVMNGDYQTSYIEVKRGSKIGEKSAWMLSLSIDVPKIDKGVDPSIIGGIDVGVKSPLVCAINNALSRYSISDNDLFHFNKKMFARRRILLRKNRHKRAGHGARNKLKPVTVLTEKSERFRKKLIERWACEIANFFIKNKVGTVQMENLESMKRREDSYFNIRLRGFWPYAEMQSKIEFKLKQYGIKIRKVAPNNTSKTCGKCGHLNNYFNFEFRKKNKFPHFKCEKCNFKEDADYNAALNISNPKLKGTKEEP

SEQ ID NO: 408 - protein, 726 aa, synthetic construct
SEVEFSHEYWMRHALTLAKRARDEREVPVGAVLVLNNRVIGEGWNRAIGLHDPTAHAEIMALRQGGLVLQNYRLADATLYVTFEPCVMCAGAMIHSRIGRVVFGVRNGKRGAAGSLMNVLNYPGMNHCVEITEGILMDECAALLCDFYRMPRQVLNAQKKAQSSINSGGSSGGSSGSETPGTSESATPEGSGGGSSGSAKNTITKALKLKIVRPYNSAEVEKIVADEKNNRERIALEKNKDKVKEACSKHLKVAAYCTTQVERNACLFCKARKLDDKFYQKLRGQFPDAVFWQEIGEIFRQLQKQAAEIYNQSLIELYYEIFIKGKGFANASSVEHYLSDVCYTRAAELFKNAAIASGLRGKVKSNFRLKELKNMRSGLPTTKSDNFPIPLVKQKGGQYAGFEISSHNGDFIIKIPFGRWQVKKEIDKYRPWEKFDFEQVRKSPKPISLLLSTRRRKRNKGWSKDEGTEAEIRKVMNGDYQTSYIEVKRGSKTGEKSAWMLSLSIDVPKIDKGVDPSIIGGIDVGVKSPLVCAINNAFSRYSISDNDLFRFNKKMFARRRILLKKNRHKRAGHGAKNKLKPITILTEKSRRFRKKLIERWACEIADFFVKNKVGTVQMENLESMKRKEDSYFNIRLRGFWPYAEMQNKIKFKLKQYGIEIRKVAPNNTSKTCSKCGHLNNYFNFEYRRKNKFPHFKCEKCNFKENADYNAALNISNPKLKSTKEEP

SEQ ID NO: 409 - protein, 726 aa, synthetic construct
SEVEFSHEYWMRHALTLAKRARDEREVPVGAVLVLNNRVIGEGWNRAIGLHDPTAHAEIMALRQGGLAMQNYRLVDATLYVTFEPCVLCAGAMVHSRIGRVVFGVRNSKRGAAGSLMNVLNHPGMNHRVEITGGILADECAALLCDFYRMPRQAFNAQKKAQSSISPGGSSGGSSGSETPGASESVTPKSSGGSSGGSAKNTITKTLKLRIVRPYNSAEVEKIVADEKNNRERIALEKNKDKVKEACSKHLKVAAYCTTQVERNACLFCKARKLDDKFYQKLRGQFPDAVFWQEIGEIFRQLQKQAAEIYNQSLIELYYAIFIKGKGFANASSVEHYLSDVCYTRAAELFKNAAIASGLRGKVKSNFRLKELRNMKSGLPTTKSDNFPIPLVRQKGGQYTGFEISNHDGDFIIKIPFGRWQVKKEINKHRPWEKFDFEQVRKSPKPISLLLSTQRRKRNKGWSKDEGTEAEIRKVMNGDYQTSYIEVKRGSKIGEKSAWMLNLSIDVPKIDKGVDPSIIGGIDVGVKSPLVCAINNAFSRYSISDNDLYRFNKKMFARRRILLKKSKHKRAGHGAKNKLKPITILTEKSGRFRKKLIERWACEIADFFIKNKVGTVQMENLEGMKRKEDSYFNIRLRGFWPYAEMQNRIEFKLKQYGIEIRKVAPNNTSKTCSKCGHLNNYFNFEYRKKNKFPHFKCEKCNFKENADYNAALNISNPKLRSTKEEP

SEQ ID NO: 410 - protein, 726 aa, synthetic construct
SEVEFSHEYWMRHALTLAKRARDEREVPVGAVLVLNNRVIGEGWNRAIGLHDPTAHAEIMALRQGGLAMQNYRLIDATLYVTFEPCAMCAGAMIHSRIGRVVFGVRNSKRGAAGSLMNVLNYPGTNHRVEITEGILADECAALLCDFYRMPRQVFNARKKAQSSINSGGSSGGSSGSETPGTSESATPKSSGGSSGGSAKNTITKALKLRIVRPYNSAEVEKIVADEKNNRERVALEKNKDKVKEACSKHLKVAAYCTTQVERNACLFCKARKLDDKFYQKLRGQFPDAVFWQELGEILRQLQKQAAEIYNQSLIELYYEIFIKGKGFANASSVEHYLSDVCYTRAAELFKNAAIASGLRGKVKSNFRLKELKNMKSGLPTTKSDNFPIPLVKQKGGQYTGFEISSHNDDFIIKIPFGRWQVKKEVDKYRPWEKFDFEQVRKSPKPISLLLSTQRRKKNKGWSKDEGTEAEIRRVMNGDYQTSYIEVKRGSKIGEKSAWMLSLSIDVPKIDKGVDPSIIGGIDVGVKSPLVCAVNNAFSRYSISDNDLFHFNKKMFARRRILLKKSKHKRAGHGAKNKLKPITILTEKSRRFRKKLIERWACEIADFFIKNKVGTVQMENLESMKRREDSYFNIRLRGFWPYAEMQNKIEFKLKQYGIEIRKVAPNNTSKTCSKCGHLNNYFNFEYRKKNKFPHFKCEKCNFKENADYNAALNISNPKLKGTKEEP

SEQ ID NO: 411 - protein, 726 aa, synthetic construct
SEVEFSHEYWMRYALTLAKRARDEREVPVGAVLVLNNRVIGEGWNRAIGLHDPTAHAEIMALRQGGLVMQNYRLTDATLYVTFEPCVMCAGAMIHSRIGRVVFGVRNSKRGAAGSLMNVLNYPGMNHCVEITEGILMDECAALLCDFYRMPRQVLNAQKKAQSSISSGGPSGGSSCSETPGASESVTPKSSGGSSTGSTKNTITKTLKLRIVRPYNSAEVEKIVADEKNSREKIALEKNKDKVKEACSEHLKVAAYCTTQVERNACPFCKARKLDDKFYQKLRGQFPDAVFWQELGEILRQLQKQAAEIYNQSLIELYYEIFIKGRGFANASSVEHYLSDVCYTRAAELFKNAAIASGLRGKVKSNFRLKELKNMKSGLPTTKSDNFPIPLVKQKGGQYTGFEISSHNDDFIIKIPFGRWQVKKEIDKYRPWEKFDFEQVRKSPRPISLLLSTQRRKRNKGWSKDEGTEAEIRKVMNGDYQTSYIEVKRGSKTGEKSAWMLNLSIDVPKIDKGVDPSIIGGIDVGVKSPLVCAINNAFSRYSISDNDLFRFNKKMFARRRILLKKNRHKRAGHGAKNKLKPISILTGKSERFRKKLIERWACEIADFFIKNKVGTVQMENLESMKRKEDSYFNIRLRGFWPYAEMQNKIEFKLKQYGIEIRKVAPNNTSKTCSKCGHLNNYFNFEYRKKNKFPHFKCEKCNFKENADYNAALNISNPKLKSTKEEP

SEQ ID NO: 412 - protein, 726 aa, synthetic construct
SEVEFSHEYWMRHALTLAKRARDEREVPVGAVLVLNNRVIGEGWNRAIGLHDPTAHAEIMALRQGGLAMRNYRLVDATLYVTFEPCVLCAGAMVHSRIGRVVFGVRNSKRGAAGSLMNVLNHPGMNHRVEITEGILVDECAALLCDFYRMPRQVFNAQKRAQSSISSGGSSGGSSGSGTPGASESVTPKSSVGSSAGSTKNTITKTLKLRIVRPYNSAEVEKIVADEKNNREKIALEKNKDKVKEACSEHLKVAAYCTTQVERNACLFCKARKLDDRFYQKLRGQFPDAVFWQEIGEIFRQLQKQAAEIYNQSLIELYYEILIKGKGFANASSVEHYLSDVCYTRAAKLFKNAAIASGLRNKIKSNFRLKELRNMKSGLPTTKSDNFPIPLVRQKGGQYTGFEISNHNSDFIIKIPFGRWQVKEEIDKYRPWEKFDFEQVRKSPKPISLLLSTQRRKKNKGWSKDEGTEAEIRRVMNGDYQTSYIEVKRGSKIGEKSAWMLNLSIDVPKIDKGVDPSIIGGIDVGVKSPLVCAINNSSSRYSICDNDLFRFNKKMFARRRILLKKNRHKRAGHGAKNKLKPITILTKKSERFRKKLIERWACEIADFFIKNKVGTVQMENLEGMKRKEDSYFNIRLRGFWPYAEMQNKIEFKLKQYGIEIRKVAPNNTSKTCSKCGHLNNYFNFEYRKKNKFPHFKCEKCNFKENADYNAALNISNPKLKSTKEEP

SEQ ID NO: 413 - protein, 726 aa, synthetic construct
SEVGFSHEYWMRHALTLAKRARDEREVPVGAVLVLNNRVIGEGWNRAIGLHDPTAHAEIMALRRGGLVMQNYRLTDATLYVTFEPCVMCAGAMIHSRIGRVVFGVRNSKRGAAGSLMNVLNYPGMNHRVEITEGILADECAALLCDYYRMPRQVFNARKKAQSSINSGGSSDGGSGSETPGTSESATPESSGGSSGVSAKNTITKTLKLRIVRPYNSTEVEKIVADEKNNREKIALEKNKDKVKEACSEHLKVAAYCTTQVERSACLFCKARKLDDKFYQKLRGQFPDAVFWQEIGEIFRQLQRQAAEIYNQSLIELYYEIFIKGKGFANASSVEHYLSDVCYTRAAELFRNAAIASGLRGKVKSNFRLKELKNMKSGLPTTKSDNFPIPLVKQKGGQYTGFEISSHNDDFIIKIPFGRWQVKKEIDKYRPWEKFDFEQVRKSPKPISLLLSTQRRKRNKGWSKDEGTEAEIRKVMNGDYQTSYIEVKRGSKIGEKSAWMLNLSIDVPKIDKGVDPSIIGGIDVGVRSPLVCAIDNAFSRYSISDNDLFHFNKKMFARRRILLKKNRHKRAGHGAKNKLKPISILTEKSKRFRKKLIERWACEIADFFIKNKVGTVQMENLESMKRREDSYFNIRLRGFWPYAEMQNKIEFKLKQYGIEIRKVAPNNTSKTCSKCGHLNNYFNFEYRKMNKFPHFKCEKCNFKENADYNAALNISNPKLRSTKEEP

SEQ ID NO: 414 - protein, 726 aa, synthetic construct
SEVEFSHEHWMRHALTLAKRARDEREVPVGAVLVLNNRVIGEGWNRAIGLHDPTAHAEIMALRQGGLVMQNYRLTDATLYVTFEPCVMCAGAMIHSRIGRVVFGVRNSKRGAAGSLMNVLNYPGMNHCVEITEGILVDECAALLCDFYRMPRQVLNAQKKAQSSINPGGSSGGSGGSETPGTSESATPESFGGSSGGSAKNTITKTLKLRIVRPHNSAEVEKIVADEKNNREKIALEKNKDKVKEACSKHLKMASYCTTQVERSACLFCKARKLDDKFYQKLRSQFPDAVFWQELGGIFRQLQKQAAEIYNQSLIELYYEIFIKGKGFANASSVEHYLSDVCYTRAAELFKNAAIASGLRGKVKSNFRLKELKNMRSGLPTTKSDNFPIPLVKQKGGQYTGFEISSHNDDFIIKIPFGRWQMKKEIDRYRPWEKFDFEQVRKSPKPISLLLSTQRRKRNKGWSKDEGTEAEIRRVMNGDYQTSYIEVKRGSKIGEKSAWMLSLSIDVPKIDKGVDPSIIGGIDVGVKSPLVCAINNAFCRYSISDNDLFHFNKKMFARRRILLKKSRHKRAGHGAKNKLKPVSILTEKSKRFRKKLIERWACEIADFFIKNKVGTVQMENLESMKRKEDSYFNIRLRGFWPYAEMQNKIEFKLKQYGIEIRKVAPNNTSKTCSKCGHLNNYFNFEYRKKNKFPHFKCEKCNFKENADYNAALNISNPKLKSTKEEP

SEQ ID NO: 415 - protein, 726 aa, synthetic construct
SEVEFSHEYWMRHALTLAKRARDEREVPVGAVLVLNNRVIGEGWNRAIGLHDPTAHAEIMALRQGGLAMQNYRLVDATLYVTFEPCVLCAGAMVHSRIGRVVFGVRNSKRGAAGSLMNVLNHPGMNHRVEITGGILVDECAALLCDFYRMPRQVLNAQKKAQSSISPGGSSGGSSGSETPGASESVTPKSSGGSSGGSAKNTITKTLKLRIVRPYNSAEVEKIVADEKNNREKIALEKNKGKVKEACSKHLEVAAYCTTQVERNACLFCKARKLDDKFYQKLRGQFPDAVFWQELGEIFRQLQRQAAEIYNQSLIELYYEIFIKGKGFANASSVEHYLSDVCYTRAAELFKNAAIASGLRGKVKSNFRLKELKNMKSGLPTTKSDNFPIPLVKQKGGQYTGFEISSHNDDFIIKIPFGRWQVRKEIDKYRPWEKFDFEQVRKSAKPISLLLSTQRRKRNKGWSKDEGTEAEIRKVMNGDYQTSYIEVKRGSKIGEKSAWMLNLSIDVPKIDKGVDPSIIGGIDVGVKSPLVCAINNAFSRYSISDNDLFRFNKKMFARRRILLKKNRHKRAGHGAKNKLKPISVLTEKSGRFRKKLIERWACEIADFFIKNKVGTVQMENLGSMKRKEDSYFNIRLRGFWPYAEMQNKIEFKLKQYGIEIRKVAPDNTSKTCSKCGHLNNYFNFEYRKKNKFPHFKCEKCNFKEDADYNAALNISNPKLKSTKEEP

SEQ ID NO: 416 - protein, 726 aa, synthetic construct
SEVEFSHEYWMRHALTLAKRARDEREVPVGAILVLNNRVIGEGWNRAIGLHDPTAHAEIMALRQGGLVMQNYRLIDATLYVTFEPCVMCAGAMIHSRIGRVVFGVRNNKHGAAGSLVNVLDYPGMNHRVEITEGILADECAALLCDFYRMPRQVFNARKKAQSSINPGGSSGGGSGSETPGTSESATPESSGGSSGSSAKNTITKTLKLRIVRPYNSAEVEKIVADEKNNREKIALEKNKDKVKEACSKHLKVAAYCTTQVERNACLFCKARKLDDKFYQKLRGQFPDAVFWQELGGIFRQLQKQAAEIYNQSLIELYYEIFIKGKGITNASSVEHYLSDVCYTRAAELFKNAAIASGLRSKVKSNFRLKELKNMKSGLPTTKSDNFPIPLVKQKGGQYTGFEISNHNSDFIIKIPFGRWQVKKEINKYRSWEKFDFEQVRKSPKPISLLLSTQRRKRNKGWSKDEGTEAEIRKVMNGDYQTSYIEVKRGSRIGEKSAWMLSLSIDVPKIDKGVDPSIIGGIDVGVKSPLVCAINNALSRYSISDNDLFHFNKKMFARRRILLKKNRHRRAGHGAKNKLKPITILTGKSERFRKKLIERWACEIADFFIKNKVGTVQMENLESMKRKEDSYFNIRLRGFWPYAEMQNKIEFKLKQYGIEIRKVAPNNTSKTCSKCGHLNNYFNFEYRKKNKFPRFKCEKCNFKEDADYNAALNISNPKLKGTKEEP

SEQ ID NO: 417 - protein, 726 aa, synthetic construct
SEVEFSHEYWMRHALTLAKRARDEREVPVGAVLVLNNRVIGEGWNRTAGLHDPTAHAEIMALRQGGLVMRNYRLTDATLYVTFEPCVMCAGAMIHSRIGRVVFGVRNSKRGAAGSLMNVLNYPGMNHCVEITEGILVDECAALLCDFYRMPRQVLNAQKKAQSSISPGGSSGGSSGSETPGASESVTPKSSGGSSGGSAKNTITKTLKLRIVRPYNSAEVEKIVADEKNNREKIALEKNRGKVKEACSKHLEVAAYCTTQVERNACLFCKARKLDDKFYQKLRGQFPDAVFWQELGGIFRQLQKQAAEIYNQSLIELYYEIFIKGKGITNASRVEHYLSDVCYTRAAELFKNAAIASGLRSKVRSNFRLKELKNMKSGLPTTKSDNFPIPLVKQKGGQYTGFEISSHNSDFIIKIPFGRWQVKEEIDKYRPWERFDFEQVRKSPKPISLLLSTQRRKKNKGWSKDEGTEAEIRRVMNGDYQTSYIEVKRGSKIGEKSAWMLNLSIDVPKIDKGVDPSIIGGIDVGVKSPLVCAINNSSSRYSICDNDLFRFNKKMFARRRILLKKNRHKRAGHGAKNKLKPITILTKKSERFRKKLIERWVCEVADFFVKNKVGTVQMENLESMKRKEDSYFNIRLRGFWPYAEMQNKIEFKLKQYGIKVRKVAPNNTSKTCSKCGHLNNYFNFEYRKKNKFPHFKCEKCNFKENADYNAALNISNPKLKSTKGEP

SEQ ID NO: 418 - protein, 726 aa, synthetic construct
SEVEFSHEYWMRHALTLAKRARDGREVPVGAVLVLNNRVIGEGWNRAIGLHDPTAHAEIMALRQGGLVMQNYRLIDATLYVTFEPCVMCAGAMVHSRIGRVVFGVRNSKRGAAGSLMNVLDYPGMGHRVEITEGVLADECAALLCDFYCMPRQVFNAQKRAQSSINSGGSSGGSSVSGTPGTSGSATPEGSGGSFGGSAKSTITKTLKLRIVRPYNSAEVEKIVADEKNNREKIALEKNKDKVKEACSKHLKVAAYCTTQVERNACLFCKARKLDDKFYQKLRGQFPDAVFWQELGEIFRQLQKQAAEIYNQSLIELYYEIFIKGKGFANASSVEHYLSDVCYTRAAELFKNAAIASGLRGKVKSNFRLKELKNMKSGLPTTKSDNFPIPLVKQKGGQYTGFEISSHNDDFIIKIPFGRWQVKEEIDKYRPWEKFDFEQVRKNPKPISLLLSTQRRKRNKGWSKDEGTEAEIRKVMNGDYQTSYIEVKRGSKIREKSAWMLNLSIDVPKIDKGVDPSIIGGIDVGVKSPLVCAINNAFSRYSISDNDLFRFNKKVFARRRILLKKNRHKRAGHGTKNKLKPITILTEKSGRFRKKLIERWACEIANFFIKNKVGTVQMENLESMKRKEDSYFNIRLRGFWPYAEMQNKIEFKLKQYGIVVRKVAPNNTSKTCSKCGHLNNYFNFEYRKKNKFPHFKCERCNFKENADYNAALNISNPKLKSTKGEP

SEQ ID NO: 419 - protein, 726 aa, synthetic construct
SEVEFSHEYWMRHALTLAKRARDGREVPVGAVLVLNNRVIGEGWNRAIGLHDPTAHAEIMALRQGGLVMQNYRLIDATLYVTFEPCVMCAGAMVHSRIGRVVFGVRNSKRGAAGSLMNVLDYPGMGHRVEITEGILADECAALLCDFYCMPRQVFNAQKRAQSSINSGGSSGGSSGSETPGASESVTPKSSGGSSGGSAKNTITKTLKLRIVRPYNSAEVEKIVADEKNNREKIALEKNKGKVKEACSKHLEVAAYCTTQVERNACLFCRARKLDDKFYQKLRGQFPDAVFWQELGEIFRQLQKQAAEIYNQSLIELYYEIFIKGKGFANASSVEHYLSDVCYTRAAELFKNAAIASGLRGKVKSNFRLKELKNMKSGLPTTKSDNFPIPLVKQKGGQYTGFEISSHNDDFIIKIPFGRWQVKKEIDKYRPWEKFDFEQVRKSPKPISLLLSTQRRKRNKGWSKDEGTEAEIRKVMNGDYQTSYIEVKRGSKIGEKSAWMLNLSIDVPKIDKGVDPSIIGGIDVGVKSPLVCAINNAFSRYSISDNDLFHFNKKMFARRRILLKKNRHKRDGHGARNKLKPITVLAEKSERFRKKLIERWACEIANFFIKNKVGTVQMENLESMKRKEDSYFNIRLRGFWPYAEMQDKIEFKLKQYGIEIRKVAPNNTSKTCSRCGHLNNYFNFEYRRKNKFPHFKCEKCNFKENADYNAALNISNPKLKSTKEEP

SEQ ID NO: 420 - protein, 726 aa, synthetic construct
SEVEFSHEYWMRHALTLAKRARDEREVPVGAILVLNNRVIGVGWNRAIGLHDPTAHAEIMALRQGGLVTQNYRLIDATLYVTFEPCVMCAGAMIHSRIGRVVFGVRNSKHGAAGSLVNVLNYPGMNHRVEITEGILADECAALLCDFYRMPRQVFNARKKAQSSINSGGSSGGSSGSETPGTSESVTPKSSGGSSAGSTKNTITKTLKLRIVRPYNSAEVEKIVADEKNSREKIALERNKDKVREACSEHLKVAAYCTTQVERNACLFCKARKLDDRFYQKLRGQFPDAVFWQETGEIFRQLQRQAAEIYNQSLIELYYEIFIKGKGFANASSVEHYLSDVCYTRAAELFKNAAIASGLRGKVKSNFRLKELKNMKSGLPTTKSDNFPIPLVKQKGGQYTGFEISSHNDDFIIKIPFGRWQVKKEIDKYRPWEKFDFEQVRKSPKPISLLLSTQRRKRNKGWSKDEGTEAEIRKVMNGDYQTSYIEVKRGSKIGEKSAWMLNLSIDVPKIDKGVDPSIIGGIDVGVRSPLVCAINNAFSRYSVSDNDLFHFNKKMFARRRILLKKNRHKRAGHGAKNKLKPITILTEKSVRFRKKLIERWACEIADFFIKNKVGTVQMENLESMKGKEDSYFNIRLRGFWPYAEMQNKIEFKLKQYGIEIRKVAPNNTSKTCSKCGHLNNYFNFEYRKKNKFPHFKCEKCHFKEDADYNAALNISNPKLRCTKEEP

SEQ ID NO: 421 - protein, 726 aa, synthetic construct
SEVEFSHEYWMRHALTLAKRARDEREVPVGAILVLNNRVIGEGWNRAIGLHDPTAHAEIMALRQGGLVMQNYRLIDATLYVTFEPCVMCAGAMIHSRIGRVVFGVRNNKHGAAGSLVNVLDYPGMNHRVEITEGILADECAALLCDFYRMPRQVFNARKKARSSISPGGSSGGSSGSETPGTSESATPESSGGSSGGSAKDTITKTLKLRIVRPYNSAEVEKIVADEKNSREKIALEKNKDKVKEACSKHLKVAAYCTTQVERNACLFCKARKLDDKFYQKLRGQFPDAVFWQETGEIFRQLQRQAAEIYNQSLIELYYEIFIKGKGFANASSVEHYLSDVCYTRAAELFKNAAIASGLRGKVKSNFRLKELKNMKSGLPTTKSDNFPIPLVKQKGGQYTGFEISSHNDDFIIKIPFGRWQVKEEISKYRPWEKFDFEQVRKSPKPISLLLSTQRRKRNKGWSKDEGTEAEIRKVMNGDYQTSYIEVKRGSRIGEKSAWMLSLSIDVPKIDRGVDPSIIGGIDVGVKSPLVCAINNALSRYSISDNDLFHFNKKMFARRRILLKKNRHRRAGHGARNKLKPITVLTEKSKRFRKKLIERWACEIANFFIKNKVGTVQMENLESMKRKEDSYFNIRLRGLWPYAEMQNKIEFKLKQYGIKIRKVAPNNTSKTCSKCGHLNNYFSFEYRKKNKFPRFKCEKCNFKEDADYNAALNISNPKLKSTKEEP

SEQ ID NO: 422 - protein, 726 aa, synthetic construct
SEVEFSHEYWMRHALILAKRARDEREVPVGAVLVLDNRVIGEGWNRAIGLHDPTAHAEIMALRQGGLVMQNYRLIDATLYVTFEPCIMCAGAMIHSRIGRVVFGVRNSKRGAAGSLMNVLNYPGMNHCVEITEGILVDECAALLCDFYRMPRQVLSAQKKAQSSISSGGSSGGSSCSETPGTSESVAPKSSGGSSAGSTKNTITKTLRLRIVRPYNSAEVEKIVADEKNSRERIALEKNKDKVKEACSEHLKVAAYCTTQVERNACLFCKARKLDDRFYQKLRGQFPDAVFWQEIGEIFRQLQKQAAEIYNQSLIELYYEIFIKGKGFANASSVEHYLSDVCYTRAAELFKNAAIASGLRGKVKSNFRLKELKNMKSGLPTTKSDNFPIPLVKQKGGQYTGFEVSSHNDDFIIKIPFGRWQVKKEIDKYRPWEKFDFEQVRKSPRPISLLLSTQRRKRNKGWSKDEGTEAEIRKVMNGDYQTSYIEVKRGSKIGEKSAWMLNLSIDVPKIDKGVDPSIIGGIDVGVKSPLVCAINNAFSRYSISDNDLFRFNKKMFARRRILLKKNRHKRAGHGAKNKLKPISILTGKSERFRKKLIERWACEIADFFIKNKVGTVQMENLESMKRKEDSYFNIRLRGFWPYAEMQNKIEFKLKQYGIKIRKVAPNNTSRTCSMCGHLNNYFSFEYRKKNKFPHFKCEKCNFKEDADYNAALNISNPKLKSTREEP

SEQ ID NO: 423 - protein, 726 aa, synthetic construct
SEVEFSHEYWMRHALTLAKRARDEREVPVGAVLVLNNRVIGEGWNRAIGLHDPTAHAEIMALRQGGLVMQNYRLVDATLYVTFEPCVLCAGAMVHSRIGRVVFGVRNSKRGAAGSLMNVLNYPGMNHRVEITEGILADECAALLCDFYRMPRQVFNAQKKARSSINSGGPSGGSSGSETPGTSESATPVSSSGSSGGSAKNTITKTLKLRIVRPYNSAEVEKIVADEKNNREKIALEKNKDRVKEACSKHLKVASYCTTQVERNACLFCKARKLDDKFYQKLRGQFPDAVFWQELGEIFRQLQKQAAEIYNQSLIELYYEIFIKGKGFANASSVEHYLSDVCYTRAAELFKNAAIASGLRGKVKSNFRLKGLKNMKSGLPTTKSDNFPIPLVKQKGGQYTGFEISSHNDDFIIKIPFGRWQVKKEIDKYRPWEKFNFEQVRKSPKPISLLLSTQRRKRNRGWSKDEGTEAEIKRVMNGDYQTSYIEVKRGSKIGEKSAWMLNLSIDVPKIDKGVDPSIIGGIDVGVKSPLVCAINNAISRYSISDNDLFHFNKKVFARRRILLKKNRHRRAGHGTKNKLKPITILTEKSKRFRKKLIERWACEIADFFIKNKVGTVQMENLESMKRKEDSYFNIRLRGFWPYAEMQNKIEFKLKQYGIKIRKVAPNNTSRTCSKCGHLNNYFSFEYRKKNKFPHFKCEKCNFKEDADYNAALNISNPKLKGTKEEL

SEQ ID NO: 424 - protein, 726 aa, synthetic construct
SEVEFSHEYWMRHALTLAKRARDGREVPVGAVLVLNNRVIGVGWNRAIGLHDPTAHAEIMALRQGGLVMQNYRLTDATLYVTFEPCVMCAGAMVHSRIGRVVFGVRNSKRGAAGSLMNVLDYPGMGHRVEITEGILADECAALLCDFYCMPRQVFNAQKKAQPSISPGGSSGGSSGSETPGASESVTPRSSGGSSGGSAKNTITKTLKLRIVRPYNSAEVEKIVADEKNNREKIALEKNKGKVKEACSKHLEVAAYCTTQVERNACLFCKARKLDDKFYQKLRGQFPDAVFWQELGEIFRQLQKQAAEIYNQSLIELYYEIFIKGKGFANASSVEHYLSDVCYTRAAELFKNAAIASGLRGKVKSNFRLKELRNMKSGLPTTKSDNFPIPLVKQKGGQYTGFEISSHNDDFIIKIPFGRWQVRKEIDKYRPWEKFDFEQVRKSPKPISLLLSTQRRKRNRGWSKDESTEAEIKKVMNGDYQTSYIEVKRGSKVGEKSAWMLNLSIDVPKIDKGVDPSIIGGIDVGVKSPLVCAINNAFSRYSISDNDLYRFNKKMFARRRILLKKSKHKRAGHGAKNKLKPITILTEKSGRFRKKLIERWACEIADFFIKNKVGTVQMENLEGMKRKEDSYFNIRLRGFWPYAEMQNKIEFKLKQYGIEIRKVAPNNTSKTCSKCGHLNNYFNFEFRKKNKFPHFKCEKCNFKEDADYNAALNISNPKLKSTKGEP

SEQ ID NO: 425 - protein, 726 aa, synthetic construct
SEVEFSHEYWMRRALTLAKRARDEREVPVGAVLVLNNRVIGEGWNRAAGLHDPTAHAEIMALRQGGLVMQNYRLIEATLYVTFEPCIMCAGAMIHSRIGRVVFGVRNSKRGAAGSLMNVLNYPGMNHRVEITEGILADECAALLCDYYRMPRQVFNARKKAQSSINSGGSSDGGSGSETPGTSESATPESSGGSSGGSAKNTITKTLKLRIVRPYNSAEVEKIVADEKNIREKIALEKNKDKVKEACSEHLKVAAYCTTQVERSACLFCKARKLDDKFYQKLRGQFPDAVFWQEIGEIFRQLQKQAAEIYNQSLIELYYEIFIKGKGFANASSVEHYLSNVCYTRAAELFKNAAIASGLRGKVKSNFRLKELKNMKSGLPTTKSDNFPIPLVKQKGGQYTGFEISSHNDDLIIKIPFGRWQVKKEIDKYRPWEKFDFEQVRKSPKPISLLLSTQRRKRNKGWSKDEGTEAEIRKVMNGDYQTSYIEVKRGSKIGEKSAWMLNLSIDVPKIDKGVDPSIIGGIDVGVKSPLVCAINNSSSRYSICDNDLFRFNKKMFARRRILLKKNRHKRAGHGAKNKLKPITILTKKSERFRKKLIERWVCEVADFFIKNKVGTVQMENLESMKRKEDSYFNIRLRGFWPYAEMQNKIEFKLKQYGIEIRRVAPNNTSRTCSKCGHLNNYFNFEYRRKYKFPHFKCEKCNFREDADYNAALNISNPKLKSTKEEP

SEQ ID NO: 426 - protein, 726 aa, synthetic construct
SEVEFSHEYWMRHALTLAKRARDEREVPVGAILVLNNRVIGEGWNRAIGLHDPTAHAEIMALRQGGLVMQNYRLIDATLYVTFEPCVMCAGAMIHSRIGRVVFGVRNSKHGAAGSLVNVLNYPGMNHRVEITEGILADECAALLCDFYHMPRQVFNARKRAQSSINSGGSSGGSSGSGTPGTSESATPKSSGGSSGGSAKNTITKALKLRIVRPYNSAEVEKIVADEKNNREKIALEKNKDKVKEACSKHLKVASYCTTQVERNACPFCKARKLDDKFYQKLRGQFPDAVFWQELGEILRQLQKQAAEIYNQSLIELYYEIFIKGRGFANAGSVEHYLSDVCYTRAAELFKNAAIASGLRGKVKSNFRLKELKNMKSGLPTTKSDNFPIPLVKQKGGQYTGFEISSHNDDFIIKIPFGRWQVKKEIDKYRPWEKFDFEQVRKSPKPISLLLSTQRRKRNKGWSKDEGTEAEIRKVMNGDYQTSYIEVKRGSKIGEKSAWMLSLSIDVPKIDKGVDPSIIGGIDVGVKSPLVCAVNNALSRYSIDDNDLFRFNKKMFARRRILLKKSRHKRAGHGAKNKLKPITILTEKSGRFRKKLIERWACEIADFFIKNKVGTVQMENLESMKRKEDSYFNIRLRGFWPYAEMQNKIEFKLKQYGIEIRKVAPNNTSRTCSKCGHLNNYFNFEYRKKNKFPHFKCEKCNFKENADYNAALNISNPKLKSTKEEP

SEQ ID NO: 427 - protein, 725 aa, synthetic construct
SEVEFSHEYWMRHALTLAKRARDEREVPVGAVLVLNNRVIGEGWNRAIGLHDPTAHAEIMALRQGGLVMQNYRLTDATLYVTFEPCVMCAGAMIYSRIGRVVFGVRNSKRGAAGSLMNVLNYPGMNHCVEITEGILVDECAALLCDFYRMPRQVLNAQKKAQSSISSGGSSGGSSGSETPGTSESATPESSGGGSSGSARDTITKTLQLRIVRPYNSAEVEKIVADEKNNREKIALEKNKDKVREACSKHLKVASYCTTQVERNACPFCKARKLDDKFYQKLRGQFPDAVFWQELGEILRQLQKQAAEIYNQSLIELYYEIFIKGRGFANASSVEHYLSDVCYTRAAELFKNAAIASGLRGKVKGNFRLKELKNMKSGLPTTKSDNFPIPLVRQKGGQYTGFEISSRNDDFIIKIPFGRWQVKKEIDKYRPWEKFDFEQVRKSPKPISLLLSTQRRKRNKGWSKDEGTEAEIRKVMNGDYQTSYIEVKRGSKTGEKSAWMLNLSIDVPKIDKGVDPSIIGGIDVGVKSPLVCAINNAFSRYSISDNDLFHFNKKMFARRRILLKKNRHKRAGHGAKNKLKPITILTEKSKRFRKKLIERWACEIADFFIKNKVGTVQMENLESMKRKEDSYFNIRLRGFWPYAEMQNKIEFKLKQYGIEIRKVAPNNTSKTCSKCGHLNNYFNFEYRKKNKFPHFKCEKCNFKENADYNAALNISNPKLKSTEKP

SEQ ID NO: 428 - protein, 725 aa, synthetic construct
SEVEFSHEYWMRHALTLAKRARDEREVPVGAVLVLNNRVIGEGWNRAVGLHDPTAHAEIMALRQGGLVMQNYRLTDATLYVTFEPCVMCAGAMIHSRIGRVVFGVRNSKRGAAGSLMNVLNYPGMNHCVEITEGILVDECAALLCDFYRMPRQVLNAQKKAQSSISSGGSSGGSSCSETPGASESVTPKSSGGGFGGSAKNTITKTLQLRIVRPYNSAEVEKIVADEKNNREKIALEKNKDKVKEACSKHLKVASYCTTQVERNACLFCKARKLDDKFYQKLRGQFPDAVFWQELGEIFRQLQKQAAEIYNQSLIELYYVIFIKGKGFANASSVEHYLSDVCYTRAAELFKNAAIASGLRGKVKSNFRLKELKNMKSGLPTTKSDNFPIPLVKQKGGQYTGFEISSHNDDFIIKIPFGRWQVKKEIDKYRPWEKFDFEQVRKSPKPISLLLSTQRRKRNKGWSKDEGTEAEIRKVMNGDYQTSYIEVKRGSKIGEKSAWMLNLSIDVPKIDKGVDPSIIGGIDVGVKSPLVCAINNAFSRYSISDNDLFHFNKKMFARRRILLKKNGHKRAGHGARNKLKPITVLTEKSKRFRKKLIERWACEIANFFIRNRVGTVQMENLESMKRKEDSYFNIRLRGFWPYAEMQNRIEFKLKQYGIEIRKVAPNNTSKTCSKCGHLNNYFSFEYRKKNKFPHFKCEKCNFKEDADYNAALNISNPKLKSTEEL

SEQ ID NO: 429 - protein, 726 aa, synthetic construct
SEVEFSHEYWMRHALTLAKRARDEREVPVGAVLVLNNRVIGEGWNRAIGLHDPTAHAEIMALRQGGLVMQNYRLTDATLYVTFEPCVMCAGAMIHSRIGRVVFGVRNSKRGAAGSLMNVLNYPGMNHCVEITEGILVDECAALLCDFYRMPRQVLSAQKKAQSSISPGGSSGGSSGSETPGASGSVTPKSSGGSSAGSTKDTITKTLKLRIVRPYNSAEVEKIVADEKNSREKIALEKNKDKVKEACSEHLKVAAYCTTQVERNACLFCKARKLDDRFYQKLRGQFPDAVFWQEIGEIFRQLQKQAAEIYNQSLIELYYEIFIKGKGFANASSVEHYLSDVCYTRAAELFKNAAIASGLRGKVKSNFRLKELKNMKSGLPTTKSDNFPIPLVKQKGGQYTGFEISNHNSDFIIKIPFGRWQAKKEIDKYRPWEKFDFEQVRKSPKPISLLLSTQRRKKNRGWSKDEGTEAEIKKVMNGDYQTSYIEVKRGSKIGEKSAWMLSLSIDVPKIDKGVDPSIIGGIDVGVKSPLVCAINNAFSRYSISDNDLFHFNKKMFARRRILLKKNRHKRAGHGAKNKLKPISILTEKSKRFRKKLIERWACEVADFFIKNKVGTVQMENLESMKRKEDSYFNIRLRGFWPYAEMQNKIEFKLKQYGIEIRKVAPNNTSKTCSKCGHLNNYFNFEYRRKNKFPHFKCEKCNFKEDADYNAALNISNPKLKSTKEEP

SEQ ID NO: 430 - protein, 726 aa, synthetic construct
SEVEFSHEYWMRHALTLAKRARDEREVPVGAVLVLNNRVIGEGWNRAIGLHDPTAHAEIMALRQGGLAMQNYRLVDATLYVTFEPCVLCAGAMVHSRIGRVVFGVRNSKRGAAGSLMNVLNHPGMNHRVEITGGILADECAALLCDFYRMPRQVFNAQKKARSNINPGGSSGGSSGSETLGTSGSVTPKSSGGSSAGSTKDTITKTLKLRIVRPYNSAEVEKVVADEKNNREKIAIEKNKDMVKEACSKHLKVASYCTTQVERNACLFCKARKLDDKFYQKLRGQFPDAVFWQELGGIFRQLQKQAAEIYNQSLIELYYEIFIKGKGITNASRVEHYLSDVCYTRAAELFKNAAIASGLRSKVRSNFRLKELKNMKSGLPTTKSDNFPIPLVKQKGGQYTGFEISSHNDDFIIKIPFGRWQVKKEIDKYRPWEKFDFGQVRKSPKPISLLLSTRRRKRNKGWSKDEGTEAEIRKVMNGDYQTSYIEVKRGSKIGEKSAWMLNLSIDVPKIDKGVDPSIIGGIDVGVKSPLVCAINNAFSRYSISDNDLFRFNKKMFARRRILLKKNRHKRAGHGAKNKLKPISILTERSERFRKKLIERWACEIADFFVKNKVGTVQMENLESMKRKEDSYFNIRLRGFWPYAEMQNKIEFKLKQYGIEIRKVAPNNTSKTCSKCGHLNNYFNFEYRKKNKFPHFKCEKCNFKENADYNAALNISNPKLKSTKGEP

SEQ ID NO: 431 - protein, 726 aa, synthetic construct
SEVEFSHEYWMRHALTLAKRARDEREVPVGAVLVLNNRVIGEGWNRAIGLHDPTAHAEIMALHQGGLVMQNYRLIDATLYVTFEPCVMCAGAMIHSRIGRVVFGARNSKRGAAGSLMNVLSYPGMNHRVEITEGILADECAALLCDYYRMPRQVFNARKKAQSGINSGGSSGGSSGSETPSASESATPESSGGSSGGSAKNTITKTLKLRIVRPYNSAEVEKIVADEKNNREKIALEKNKDKVKEACSKHLKVAAYCTTQVERNACLFCKARKLDDKFYQKLRGQFPDAVFWQEIGEIFRQLQKQAAEIYNQSLIELYYEIFIKGKGFANASSVEHYLSDVCYTRAAELFKNAAIASGLRNKIKSNFRLKELRNMKSGLPTTKSDNFPIPLVRQKGGQYTGFEISNHNGDFIIKIPFGRWQVKEEIDKYRPWEKFDFEQVRKSPKPISLLLSTQRRKKNKGWSKDEGTEAEIRRVMNGDYQTSYIEVKRGSRIGEKSAWMLSLSIDVPKIDRGVDPSIIGGIDVGVKSPLVCAINNALSRYSISDNDLFHFNKKMFARRRILLKKNRHKRAGHGAKNKLKPITIMTEKSKRFRKKLIERWACEIADFFIKNKVGTVQMENLESMKRKEDSYFNIRLRGFWPYAEMQNKIEFKLKQYGIEIRKVAPNNTSKTCSKCGHLNNYFNFEYRKKNKFPHFKCEKCNFKEDADYNAALNISNPKLKSTKEEP

SEQ ID NO: 432 - protein, 726 aa, synthetic construct
SEVEFSHEYWMRHALTLAKRARDEREVPVGAVLVLNNRVIGEGWNRAIGLHDPTAHAEIMALRQGGLVMQNYRLVDATLYVTFEPCVLCAGAMVHSRIGRVVFGVRNSKRGAAGSLMNVLNYPGMNHRVEITEGILADECAALLCDFYRMPRQVFNARKKAQSSINPGGSSGGSSGSGTPGTSESATPESSGGSSSGSAKNTITKTLKLRIVRPYNSAEVEKIVADEKNNREKIALEKNKDKVKEACSKHLKVAAYCTTQVERNACLFCKARKLDDKFYQKLRGRFPDAVFWQEISEIFRQLQKQAAEIYNQSLIELYYEIFIKGKGFANASSVEHYLSDVCYTRAAELFKNAAIASGLRGKVKSNFRLKELKNMKSGLPTTKSDNFPIPLVKQKGGQYTGFEISSHNDDFIIKIPFGRWQVKKEIDKYRPWEKFDFEQVRKSPKPISLLLSTQRRKRNKGWSKDEGTEAEIRKVMNGDYQTSYIEVKRGSKIGEKSAWMLNLSIDVPKIDKGVDPSIIGGIDVGVKSPLVCAINNTFSRYSISDNDLFRFNKKMFARRRILLGKNRHKRAGHGVKNKLKPITILTEKSKRFRKKLIERWACEIADFFIKNKVGTVQMENLESMKRREDSYFNIRLRGFWPYAEMQNKIEFKLKQYGIVVRKVAPNNTSKTCSKCGHLNNYFNFEYRKKNKFPHFKCEKCNFKEDADYNAALNISNPKLKSTKGEP

SEQ ID NO: 433 - protein, 726 aa, synthetic construct
SEVEFSHEYWMRRALTLAKRARDEREVPVGAVLVLNNRVIGVGWNRAVGLHDPTAHAEIMALRQGGLVMQNYRLIDATLYVTFEPCVMCAGAMIHSRIGRVVFGVRNNKHGAAGSLMNVLNYPGMNHRVEITEGILADECAALLCDFYRMPRQVFNARKKAQSSINPGGSSGGSGGSETPGTSESATPENSGGSSGSSAKNTITKTLKLRIVRPYNSAEVEKIVADEKNSREKIALEKNKDKVKEACSKHLKVASYCTTQVERNACLFCKARKLDDKFYQKLRGQFPDAVFWQELGEIFRQLQKQAAEIYNQCLIELYYEIFIKGKGFANASSVEHYLSDVCYTRAAELFKNAAIASGLRGKVKSNFRLKELKNMKSGLPTTKSDNFPIPLVKQKGGQYTGFEISSHNDDFIIKIPFGRWQAKKEIDKYRPWEKFDFEQVRKSPKPISLLLSTQRRKRNKGWSKDEGTEAEIRKVMNGDYQTSYIEVKRGSKTGEKSAWMLSLSIDVPKIDKGVDPSIVGGIDVGVKSPLVCAINNALGRYSISDNDLFHFNKKMFARRRILLKKNGHKRAGHGAKNKLKPITIMTEKSKRFRKKLIERWACEIADFFVKNKVGTVQMENLESMKRKEDSYFNIRLRGFWPYAEMQSKIEFKLKQYGIKIRKVAPNNTSKTCSKCGHLNNHFSFEYRKKNKFPHFKCEKCNFKEDADYNAALNISNPKLKSTKEEP

SEQ ID NO: 434 - protein, 726 aa, synthetic construct
SEVEFSHEYWMRHALTLAKRARDEREVPVGAVLVLNNRVIGEGWNRAIGLHDPTAHAEIMALRQGGLVMQNYRLIDATLYVTFEPCVMCAGAMIHSRVGRVVFGVRNSKHGAAGSLMNVMNYPGMNHRVEITEGILADECAALLCDFYRMPRRVFNARKKAQSSIDPGGPSGGSSGSETPGTSESATPESSGGSSGGSAKNTITKTLKLRIVRPYNSTEVEKIVADEKNNREKIALEKNKDKVKEACSKHLKVASYCTTQVERNACLFCRARKLDDKFYQKLRGQFPDAVFWQELGEIFRQLQKQAAEIYNQSLIELYYEIFIKGKGFANASSVEHYLSDVCYTRAAELFKNAAIASGLRGKVKSNFRLKELKNMKSGLPTTKSDNFPIPLVKQKGGQYTGFEISSHNDDFIIKIPFGRWQVKEEIDKYRPWEKFAFEQVRKNPKPISLLLSTQRRKRNKGWSKDEGTEAEIRKVMNGDYQTSYIEVKRGSRIGEKSVWMLNLSIDVPKIDKGVDPSIIGGIDVGVKSPLVCAINNAFSRYSISDNDLFHFNKKMFARRRILLKKNRHKRAGHGAKNKLKPISILTEKSKRFRRKLIERWACEIADFFIKNKVGTVQMENLESMKRKEDSYFNIRLRGFWPYAEMQNRIEFKLKQYGIEIRKVAPNNTSKTCSKCGHLNNYFNFEYRKMNKFPHFKCEKCNFKENADYNAALNISNPKLKSTKEEP

SEQ ID NO: 435 - protein, 726 aa, synthetic construct
SEVEFSHEYWMRHALTLARRARDEREVPVGAILVLNNRVIGEGWNRANGLHDPTAHAEIMALRQGGLVMQNYRLIEATLYVTFEPCIMCAGAMIHSRIGRVVFGVRNSKRGAAGSLMNVLNYPGMNHRVEITEGILADECAALICDYYRMPRQVFNARKKAQPSINSGGSSDGGSGSETPGTSESATPESSGGSSGGSAKNTITKTLRLRIVRPFNSAEVEKIVADEKNNREKIALEKNKDKVKEACSEHLKVAAYCTTQVERSACLFCKARKLDDKFYQKLRGQFPDAVFWQEIGEIFRQLQKQAAEIYNQSLIELYYEIFIKGKGFANASSVEHYLSDVCYTRAAELFKNAAIASGLRGKVKSNFRLKELKNMKSGLPTTKSDNFPIPLVKQKGGQYTGFEISSHNDDFIIKIPFGRWQVKKEIDKYRPWEKFDFEQVRKSPKPISLLLSTQRRKRNKGWSKDEGTEAEIRKVMNGDYQTSYIEVKRGSKIGEKSAWMLSLSIDVPKIDKGVDPSIIGGIDVGVRSPLVCAINNAFSRYSISDNDLFRFNKKMFARRRILLKRNRHKRAGHGAKNKLKPITTLTEKSRRFRKKLIERWACEIADFFIKNKVGTVQMESLESMKRREDSYFNVRLRGFWPYAEMQNKIEFKLKQYGIKIRKVAPNNTSKTCSMCGHLNNYFSFEYRKKYKFPHFKCEKCNFKENADYNAALNISNPKLKSTKEEP

SEQ ID NO: 436 - protein, 726 aa, synthetic construct
SEVEFSHEYWMRHALSLAKRARDEREVPVGAVLVLNNRIIGEGWNRAIGLHDPTAHAEIMALRQGGLVMQNYRLTDATLYVTFEPCVMCAGAMIHSRIGRVVFGVRNSKRGAAGSLMNVLNYPGMNHRVEITEGILVDECAALLCDFYRMPCQVLNAQKKAQSSISSGGSSGGSSGGDTLGASESVTPKSSVGSSASSTKNTITKTLKLRIVRPYNSAEVEKIVADEKDNREKIALEKNKDKVKEACSKHLKVAAYCTTQVERNACLFCKARKLDDKFYQKLRGQFPDAVFWQEIGEIFRQLQKQAAEIYNQSLIELYYEIFIKGKGFANASSVEHYLSDVCYTRAAGLFKNAAIASGLRGKVKSNFRLKELKNMKSGLPTTKSDNFPIPLVRQKGGQYTGFEISNHDGDFIIKIPFGRWQVKKEIDKYRPWEKFDFEQVRKSPKPISLLLSTQRRKRNKGWSKDEGTEAEIRKVMNGDYQTSYIEVKRGSKIGEKSAWMLSLSIDVPKIDKGVDPSIIGGIDVGVKSPLVCAINDALSRYSISDNDLFHFNKKMFARRRILLKKNRHKRAGHGAKNKLKPISILTGKSERFRKKLIERWACEIADFFIKNKVGTVQMENLESMKRKEDSYFNIRLRGFWPYAEMQNKIEFKLKQYGIEIRKVAPNNTSKTCSKCGHLNNYFNFEYRKKNKFPHFKCEKCNFKENADYNAALNISNPKLKSTKEKP

SEQ ID NO: 437 - protein, 726 aa, synthetic construct
SEVEFSHEYWMRHALTLARRARDEREVPVGAVLVLNNRVIGEGWNRAIGLHDPTAHAEIMALRQGGLVMRNYRLIDATLYVTFEPCVMCAGAMIHSRISRVVFGVRNSKRGAAGSLMNVLNYPGMNHRVGITEGILADECAALLCDFYRMPRRVLNAQKKAQSSINSGGSSGGSSGSGTPGTSESATPESSGGSSGRSAKNTITKTLKLRIVRPYNSAEVEKIVADEKDNREKIALEKNKGKVKEACSKHLKVAAYCTTQVERNACLFCRARKLDDKFYQRLRGQFPDAVFWQETGEIFRQLQRQAAEIYNQSLIELYYEIFIKGKGFANASSVEHYLSDVCYTRAAELFKNAAIASGLRGKVKGNFRLKELKNMKSGLPTTKSDNFPIPLVKQKGGQYTGFEISNHNGDFIIKIPFGRWQVKKEINKYRPWEKFDFEQVRKSPKPISLLLSTQRRKRNKGWSKDEGTEAEIKKVMNGDYQISYIEVKRGSKIGEKSAWTLNLSVDVPKIDKGVDPSIIGGIDVGVKSPLVCAINNALSRYSISDNDLFHFNKKMFARRRILLRKNRHKRAGHGAKNKLKPISILTEKSRRFRKKLIERWACEIADFFIKNKVGTVQMEDLESMKRRGDSYFNIRLRGLWPYAEMQNKIEFKLKQYGIEIRKVAPNNTSKTCSKCGHLNNYFNFEYRKKNKFPHFKCEKCNFKENADYNAALNISNPKLKNTKEEP

SEQ ID NO: 438 - protein, 726 aa, synthetic construct
SEVEYSHEYWMRHALTLAKRARDEREVPVGAVLVLNNRVIGEGWNRAIGLHDPTAHAEIMALRQGGLVMQNYRLTDATLYVTFEPCVMCAGAMIHSRIGRVVFGVRNSKRGAAGSLMNVLNHPGMNHRVEITEGILVDECAALLCDFYRMPCQVLNAQKKAQSSISSGGSSGGSSGGDTLGASESVTPKSSGGSSGGSAKNTITKALKLRIVRPYNSAEVEKIVADEKNNRERIALEKNKDKVKEACSKHLKVATYCTTQVERNACLFCKARRLDDKFYQKLRDQFPDAVFWQEIGEIFRQLQKQAAEIYNQSLVELYYEILIKGKGIANASSVEHYLSDVCYTRAAELFKNAAIASGLRNKIKSNFRLKELRNMKSGLPTTKSDNFPIPLVRQKGGQYTGFGISNHNGDFIIKIPFGRWQVKKEIDRYRPWEKFDFEQVRKSPKPISLLLSTQRRKRNKGWSKDEGTEAEIRKVMNGDYQTSYIEVKRGSKIGEKSAWMLNLSIDVPKIDKGVDPSIIGGIDVGVKSPLVCAINNAFSRYSISDNDLFRYNKKMFARRRILLKKNRHKRAGHGARNKLKPISILTEKSKRFRKKLIERWACEIADFFIKNKVGTVQIENLESMKRREDSYFNIRLRGFWPYAEMQNKIEFKLKQYGIEIRKVAPNNTSKTCSKCGHLNSYFNFEYRKKNKFPHFKCEKCNFRENADYNAALNISNPKLRSTKEEP

SEQ ID NO: 439 - protein, 726 aa, synthetic construct
SEVEFSHEYWMRHALTLAKRARDEREVPVGAVLVLNNRVIGEGWNRAIGLHDPTAHAEIMALRQGGLVMQNYRLTDATLYVTFEPCVMCAGAMIHSRIGRVVFGVRNSKRGAAGSLMNVLNYPGMNHCVEITEGILVDECAALLCDFYRMPRQVLNAQKKAQSSISSGGSSGGSSCSETPGSSESATPESSGGGSSGSAKNTITKTLQLRIVRPYNSAEVEKIVADEKNNREKIALEKNKDKVKEACSKHLKVASYCTTQVERNACPFCKARKLDDKFYQKLRGQFPDAVFWQELGEILRQLQKQAAEIYNQSLIELYYEIFIKGRGFANAGSVEHYLSDVCYTRAAELFKNAAIASGLRGKVKSNFRLKELKNMKSGLPTTKSDNFPIPLVKQKGGQYTGFEISSHNDDFIIKIPFGRWQVKKEIDKYRPWEKFDFEQVRKSPKPISLLLSTQRRKKNKGWSKNEGTEAEIRRVMNGDYQTSYIEVKRGSKIGEKSAWMLNLSIDVPKIDKGVDPSIIGGIDVGVKSPLVCAINNAFSRYSISDNDLFRFNKKVFARRRILLKKNRHKRAGHGTKNKLKPISILTGKSERFRKKLIERWACEIADFFIKNKVGTVQMENLESMKRKEDSYFNIRLRGFWPYAEMQNRIEFKLKQYGIEIRKVAPNNTSKTCSKCGHLNNYFNFEYRKKNKFPHFKCEKCNFKENADYNAALNISNPKLKSTKEEP

SEQ ID NO: 440 - protein, 726 aa, synthetic construct
SEVEFSHEYWMRHALTLAKRARDEREVPVGAILVLNNRVIGEGWNRAIGLHDPTAHAEIMALRQGGLVMQNYRLIDATLYVTFEPCVMCAGAMIHSRIGRVVFGVRNNKHGAAGSLVNVLNYPGMNHRVEITEGILADECAALLCDFYRMPRQVFNARKKAQSSINPGGSSGGSSGSETPGASGSVTPKSSGGSSAGSTKDTITKTLKLRIVRPYNSAEVEKIVADEKNNREKIALEKNKGKVKEACSKHLKVASYCTTQVERNACLFCKARKLDDKFYQKLRGQFPDAVFWQELGGIFRQLQKQAAEIYNQSLIELYYEIFIKGRGFANASSVEHYLSDVCYTRAAELFKNAAIASGLRGKVKSNFRLKELKNMKSGLPTTKSDNFPIPLVKQKGGQYTGFEISSHNDDFIIKIPFGRWQVKKEIDKYRPWEKFDFEQVRKSPKPISLLLSTQRRKRNKGWSKDEGTEAEIKRVMNGDYQISYIEVKRGSKIGEKSAWMLSLSVDVPKIDKGVDPSIVGGIDVGVKSPLVCAIDNALSRYSISDNDLFHFNKKMFARRRILLKKNRHRRAGHGAKNKLKPISILTEKSKRFRKKLIERWACEIAGFFIKNKVGTVQMENLESMKRKEDSYFNIRLRGFWPYAEMQNKIEFKLKQYGIEIRKVAPNNTSKTCSKCGHLNNYFNFEYRKKNKFPHFKCERCNFKENADYNAALNISNPKLKSTKGEP

SEQ ID NO: 441 - protein, 726 aa, synthetic construct
SEVEFSHEYWMRHALTLAKRARDKHEVPVGAVLVLNNRVIGEGWNRAIGLHDPTAHAEIMALRQGGLVMQNYRLTDATLYVTFEPCVMCAGAMIHSRIGRVVFGVRNSKRGAAGSLMNVLNYPGMNHCVEITEGILVDECAALLCDFYRMPRQVLNAQKKAQSSISSGGSSGGSSGSETPGASGSVTPKSSGGSSAGPTKDTITKTLKLRIVRPYNSAVVEKIVADEKNSREKIALERNRDKVKEACSEHLRVAAYCTTQVERNACLFCKARKLDDKFYQKLRGQFPDAVFWQEIGEIFRQLQKQAAEIYNQSLIELYYEIFIKGKGFANASSVEHYLSDVCYTRAAELFKNAAIASGLRGKVKSNFRLKELKSMKSGLPTTKSDNFPIPLVKQKGGQYTGFEISSHNDDFIIKIPFGRWQVKKEIDKYRPWEKFDFEQVRKSPKPISLLLSTQRRKRNKGWSKDEGTEAEIRKVMNGDYQTSYIEVKRGSKTGEKSAWMLNLSIDVPKIDKGVDPSIIGGIDVGVKSPLVCAINNAFSRYSIGDNDLFHYNKKMFARRRILLKKNRHKRAGHGAKNKLKPISILTEKSKRFRKKLIERWACEIADFFIKNKVGTVQIENLESMKRKEDSYFNIRLRGFWPYAEMQNKIEFKLKQYGIEIRKVAPNNTSKTCSKCGHLNSYFNFEYRKKNKFPHFKCEKCNFKENADYNAALNISNPKLKSTKEEP

SEQ ID NO: 442 - protein, 726 aa, synthetic construct
SEVEFSHEYWMRRALTLAKRARDEREVPVGAVLVLNNRVIGEGWNRAIGLHDPTAHAEIMALRQGGLVMQNYRLTDATLYVTFEPCVMCAGAMIHSRIGRVVFGVRNSKRGAAGSLMNVLNYPGMNHCVEITEGILVDECAALLCDFYRMPRQVLSAQKKAQSSISPGGSSGGSSGSVTPGASESVTPKSSGGGSAGSTKNTITKTLKLRIVRPYNSAEVEKIVADEKNSREKTALEKNKDKVKEACSKHLKVAAYCTTQVERNACLFCKARKLDDRFYQKLRGQFPDAVFWQEIGEIFRQLQKQAAEIYNQSLIELYYEIFIKGKGFANASSVEHYLSDVCYTRAAELFKNAAIASGLRGKVKSNFRLKELKNMRSGLPTTKSDNFPIPLVKQKGGQYTGFEVSSHNDDFIIKIPFGRWQVKEEIDKYRPWEKFDFEQVRKSPKPISLLLSTQRRKKNKGWSKDEGTEAEIRRVMNGDYQTSYIEVKRGSKIGEKSAWMLNLSIDVPKIDKGVDPSIIGGIDVGVKSPLVCAINNAFSRYSISDNDLFRFNKKVFARRRILLKKNRHKRAGHGTKNKLKPISILTEKSKRFRKKLIERWACEIADFFIKNKVGTVQMENLESMKRKEDSYFNIRLRGLWPYAEMQNKIEFKLKQYGIEIRKVAPNNTSKTCSKCGHLNNYFNFEYRKKNKFPRFKCEKCNFKEDADYNAALNISNPKLKSTKEEP

SEQ ID NO: 443 - protein, 726 aa, synthetic construct
SEVEFSHEYWMRHALTLAKRARDEREVPVGAILVLNNRVIGEGWNRAIGLHDPTAHAEIMALRQGGLVMQNYRLIDATLYVTFEPCVMCAGAMIHSRIGRVVFGVRNNKHGAAGSLVNVLNYPGMSHRVEITEGILADECAALLCDFYRMPRQVFNARKKAQSSINPGGSSGGSSGSETPGTSENATPESSGGSSGSSAKNTITKTLKLRIVRPYNSAEVEKIVADEKNNREKIALEKNKDKVKEACSKHLKVAAYCTTQVERNACLFCKARRLDDKFYQKLRGQFPDAVFWQEIGEIFRQLQKQAAEIYNQSLIELYYEIFIKGKGFANASSVEHYLSDVCYTRAAELFKNAAIASGLRGKVKSNFRLKELKNMKSGLPTTKSDNFPIPLVKQKGGQYTGFEISSHNDDFIIKIPFGRWQVKKEIDKYRPWEKFDFEQVRKSPKPISLLLSTQRRKRNKGWSKDEGTEAEIRKVMNGDYQTSYIEVKRGSKIGEKSAWMLNLSIDVPKIDKGVDPSIIGGIDVGVKSPLVCAINNAFSRYSIGDNDLFRFNKKMFARRRILLKKNRHRRAGHGAKNKLKPITILTEKSVRFRKKLIERWACEIADFFIKNKVGTVQMENLESMKRKEDSYFNIRLRGFWPYAEMQNKIEFKLKQYGIEIRRVAPNNTSRTCSKCGHLNNYFNFEYRRKNKFPHFKCEKCNFKEDADYNAALNISNPKLKSTKEEP

SEQ ID NO: 444 - protein, 726 aa, synthetic construct
SEVEFSHEYWMRHALTLAKRARDEREVPVGAILVLNNRVIGEGWNRAIGLHDPTAHAEIMALRQGGLVMQNYRLTDATLYVTFEPCVMCAGALIHSRIGRVVFGVRNSKHGAAGSLVNVLNYPGMNHRVEITEGILADECAALLCDFYRMPRQVFNARKKAQSSINPSGSSGGSSGSVTPGTSESATPESSGGSSGGSAKNTITKTLKLRIVRPYNSAEVEKIVADEKNNREKIALEKNKDRVKEACSEHLKVAAYCTTQVERSACLFCKARKLDDKFYQRLRSQFPDAVFWQEIGEIFRQLQKQAAEIYNQSLIELYYEIFIKGKGIANASSVEHYLSDVCYTRAAELFKNAAIASGLRNKVKSNFRLKELRSMKSGLPTTKSDNFPIPLVRQKGGQYTGFEISNHNSDFIIKVPFGRWQVKREINKHRPWEKFDFEQVRKSPKPISLLLSTQRRKRNKGWSKDEGTEAEIRKVMNGDYQTSYIEVKRGSKIGEKSAWMLNLSIDVPKIDKGVDPGIIGGIDVGVKSPLVCAINNASSRYSISDNDLFHFNKKMFARRRILLKKNRHKRAGHGAKNKLKPITIMTEKSKRFRKKLIERWACEIADFFIKNKVGTVQMENLESMKRKEDSYFNIRLRGFWPYAEMQNKIEFKLKQYGIEIRKVAPNNTSKTCSKCGHLNNYFNFEYRKKNKFPHFKCEKCNFKENADYNAALNISNPKLKSTKEEP

SEQ ID NO: 445 - protein, 726 aa, synthetic construct
SEVEFSHEYWMRHALTLAKRARDEREVPVGAILVLNNRVIGEGWNRTTGLHDPTAHAEIMALRQGGLVVRNYRLTDATLYVTFEPCVMCAGAMIHSRIGRVVFGVRNSKRGAAGSLMNVLNYPGMNHCVEITEGILVDECAALLCDFYRMPRQVLNAQKKAQSSISPGGSSGGSSGSETPGASESVTPKSSGGSSGGSAKNTITKTLKLRIVRPYNSAEVEKIVADEKNNREKIALEKNKGKVKEACSKHLEVAAYCTTQVERNACLFCKARKLDDKFYQKLRGQFPDAVFWQELGEIFRQLQKQAAEIYNQSLIELYYEIFIKGKGFANASSVEHYLSDVCYTRAAELFKNAAIASGLRGKVKSNFRLKELKNMKSGLPTTKSDNFPIPLVKQKGGQYTGFEISSHNDDFIIKIPFGRWQVKEEIDKYRPWEKFDFEQVRKSPKPISLLLSTQRRKRSKGWSKDEGTEAEIRKVMNGDYQTSYIEVKRGSKTGEKSTWMLNLSIDVPKIDKGVDPSIIGGIDVGVKSPLVCAINNAFSRYSISDNDLFRFNKKMFARRRILLKKNRHKRAGHGAKNKLKPISILTGKSERFRKKLIERWACEIADFFIKNKVGTVQMENLESMKRKEDSYFNIRLRGFWPYAEMQNKIEFKLKQYGIEIRKVAPNNTSKTCSKCGHLNNYFNFEYRKKNKFPPFKCEKCNFMENADYNAALNISNPKLKSTKEEP

SEQ ID NO: 446 - protein, 726 aa, synthetic construct
SEVEFSHEYWMRHALTLAKRARDEREVPVGAILVLNNRVIGVGWNRAIGLHDPTAHAEIMALRQGGLVMQNYRLTDATLYVTFEPCVMCAGAMIHSRIGRVVFGVRNSKRGAAGSLMNVLNYPGMNHCVEITEGILADECAALLCDFYRMPRQVFNARKKAQSSINPSGSSGGSSGSVTPGTSESATPESSGGGFGGSAKNTITKTLKLRIVRPYNSAEVEKIVADEKDSREKIALEKNKDKVKEACSKHLKVASYCTTQVERNACLFCKARKLDDKFYQKLRGQFPDAVFWQELGGIFRQLQKQAAEIYNQSLIELYYEIFIKGKGITNASRVEHYLSDVCYTRAAELFKNAAIASGLRSKVRSNFRLKELKNMKSGLPTTKSDNFPIPLVKQKGGQYTGFEISSHNSDFIIKIPFGRWQVKEEVDKYRPWEKFDFEQVRKNPKPISLLLSTQRRKRNKGWSKDEGTEAEIRKVMNGDYQTSYIEVKRGSKIGEKSAWMLNLSIDVPKIDKGVDPSIIGGIDVGVKSPLVCAINNAFSRYSISDNDLFRFNKKVFARRRILLKKNRHKRAGHGTKNKLKPITILTEKSGRFRRKLIERWACEIANFFIKNKVGTVQMENLESMKRKEDSYFNIRLRGFWAYAEMQSKIEFKLKQYGIVVRKVAPNNTSKTCSKCGHLNNYFNFEYRKKNKFPHFKCEKCNFKENADYNAALNISNPKLKSTKGGP

SEQ ID NO: 447 - protein, 726 aa, synthetic construct
SEVEFSHEYWMRHALTLAKRARDEREVPVGAILVLNNRVIGEGWNRAIGLNDPTAHAEIMALRQGGLVMQNYRLIDATLYVTFEPCVMCAGAMIHSRIGRVVFGVRNNKHGAAGSLMNVLNYPGMNHRVEITEGILADECAALLCDFYRMPRQVFNARKKAQSSINPGGSSGGSGGSETPGTSGSATPENSGGSSGSSAKNTITKTLKLRIVRPYNSAEVEKIVADEKNNREKIALEKNKDKVKEACSKHLKVAAYCTTQVERNACLFCKARRLDDKFYQKLRGRFPDAVFWQEIGEIFRQLQKQAAEIYNQSLVELYYEILIKGKGIANASSVEHYLSDVCYTRAAELFKNAAIASGLRNKIKSNFRLKELRNMKSGLPTTKSDNFPIPLVKQKGGQYTGFEISSHNDDFIIKIPFGRWQVKKEIDKYRPWEKFDFEQVRKSPKPISLLLSTQRRKRNKGWSRDEGTEAEIKKVMNGDYQTSYIEVKRGSKIGEKSTWMLNLSIDVPKIDKGVDPSIIGGIDVGVKSPLICAINNAFSRYGISDNDLFRFNKKVFARRRILLKKNRHRRAGHGAKNKLKPITILTEKSKRFRKKLIERWACEIADFFIKNKVGTVQMENLESMKRKEDSYFNIRLRGFWPYAEMQNKIEFKLKQYGIKVRKVAPNNTSKTCSKCGHLNNYFNFEYRRKNKFPHFKCEKCNFKEDADYNAALNISNPKLKSTKEEP

SEQ ID NO: 448 - protein, 726 aa, synthetic construct
SEVEFSHEYWMRHALTLAKRARDEREVPVGAVLVLNNRAIGEGWNRAIGLHDPTAHAEIMALRQGGLVMQNYRLTDATLYVTFEPCVMCAGAMIHSRIGRVVFGVRNSKRGAAGSLMNVLNYPGMNHCVEITEGILVDECAALLCDFYRMPRQVLNAQKKAQSSISSGGSSGGSSGSETPGASGSVIPKSSGGSSAGSTKDTITKTLKLRIVRPYNSAEVEKVVADEKNNREKIAMEKNKDKVKEACSKHLKVASYCTTQVERNACLFCKARKLDDKFYQKLRGQFPDAVFWQELGGIFRQLQKQAAEIYNQSLIELYYEIFIKGKGITNAGRVEHYLSDVCYTRAAELFKNAAIASGLRSKVRSNFRLKELKNMKSGLPTTKSDNFPIPLVKQKGGQYTGFEISSHNGDFIIKIPFGRWQEKEEIDKYRPWEKFDFEQVRRSPKPISLLLSTQRRKRNKGWSKDEGTEAEIRRVMNGDYQTSYIEVKRGSKIGEKSAWMLNLSIDVPKIDKGVDPSIIGGIDVGVKSPLVCAINNAFSRYSISDNDLFRFNKKMFARRRILLKKNRHKRAGHGAKNKLKPISILTEKSKRFRKKLIERWACEIADFFIKNRVGTVQMENLESMKRKEDGYFNIRLRGFWPYAEMQNKIEFKLKQYGIEIRKVAPNNTSKTCSKCGHLNNYFNFEYRKTNKFPHFKCEKCNFKEDADYNAALNISNPKLKSTKEEP

SEQ ID NO: 449 - protein, 726 aa, synthetic construct
SEVEFSHEYWMRHALTLAKRARDEREVPVGAVLVLNNRVIGEGWNRAIGLHDPTAHAEIMALRQGGLVMQNYRLIDATLYVTFEPCVMCAGAMIHSRIGRVVFGVRNNKHGAAGSLVNVLNYPGMNHRVEITEGILADECAALLCDFYRMPRQVFNARKKARSNINSGGSSGGSSGSETPGTSESATPESSGGSSGGSAKNTITKTLTLRIVRPYNSAEVEKIVADEKNNREKIALEKNKDKVKEACSEHLKVATYCTTQVERNACPFCKARKLDDGFYQKLRGQFPDAVFWQEIGEIFRQLQKQAAEIYNQSLIELYYEIFIKGKGFANASSVEHYLSDVCYTRAAEQFKNAAIASGLRGKVKSNFRLKELKNMKSGLPTTKSDNFPIPLVKQKGGQYTGFEISSHNDDFIIKIPFGRWQVKEEIDKYRPWEKFDFEQVRKNPKPISLLLSTQRRKRNKGWSKDEGTEAEIRKVMNGDYQTSYIEVKRGSKIGEKSAWMLNLSIDVPKIDKGVDPSIIGGIDVGVKSPLVCAVNNALSRYSISDNDLFHFNKKMFARRRILLRKNRHKRAGHGAKNKLKPISTLTGKCERFRKKLIERWACEIADFFIKNKVGTVQMENLESMKRKEDSYFNIKLRGFWPYAEMQNKIEFKLKQYGIKVRRVAPNNTSKTCSKCGHLNNYFSFEYRKKNKFPHFKCEKCNFKENADYNAALNISNPKLKSTKEEP

SEQ ID NO: 450 - protein, 726 aa, synthetic construct
SEVEFSHEYWMRHALTLAKRARDEREVPVGAVLVLNNRVIGEGWNRAIGLHDPTAHAEIMALRQGGLVMQNYRLVDATLYVTFEPCVLCAGAMVHSRIGRVVFGVRNSKRGAAGSLMNVLNYPGMNHRVEITEGILADECAALLCDFYRMPRQVLNAQKKAQSSISPGGSSGGSSGSETPGASESVTPKSSGGSSGGSTKNTITKTLKLRIVRPYNSAEVEKIVADEKNNREKIALEKNKGKVKEACSKHLEVAAYCTTQVERSACLFCKARKLDDKFYQKLRGQFPDAVFWQEIGEIFRQLQKQAAEIYNQSLIELYYEIFIKGKGIANASSVGHYLSDVCYTRAAELFKNAAIASGLRSKIKSNFRLKELRNMRGGLPTTKSDNFPIPLVKQKGGQYTGFEISSHNDDFIIKIPFGRWQVKKEIDKYRPWEKFDFEQVRKSPKPISLLLSTQRRKRNKGWSKDEGTEAEIRKVMNGDYQTSYIEVKRGSKIGEKSAWMLSLSIDVPKIDKGVDPSIIGGIDVGVKSPLVCAINNAFCRYSISDNDLFHFNKKMFARRRILLKKSRHKRAGHGAKNKLKPISILTEKSKRFRKKLIERWACEIADFFIRNKVGTVQMENLESMKRKEDSYFNIRLRGFWPYAEMQNKIEFKLKQYGIEIRKVAPNNTSKTCSKCGHLNNYFNFEYRKKNKFPHFKCEKCNFKENADYNAALNISNPKLKSTKEEP

SEQ ID NO: 451 - protein, 726 aa, synthetic construct
SEVEFSHEYWMRHALTLAKRARDEREVPVGAVLVLNNRVIGEGWNRAIGLHDPTAHAEIMALRQGGLVMQNYRLADATLYVTFEPCVLCAGAMVHSRIGRVVFGVRNSKRGAAGSLMNVLNYPGMNHRVEITEGILADECAALLCDFYRMPRQVFNARKKAQSSISPGGSSGGSRGSETPGTSESATPESSGGSSGGSAKNTITKTLKLRIVRPYNSAEVEKIVADEKNNREKIALEKNKDKVQEACSKHLKVASYCTTQVERNACLFCKARKLDDKFYQKLRGQFPDAVFWQELGEIFRQLQKQAAEIYNQSLVELYYEIFIKGRGFANASSVEHYLSDVCYTRAAELFKNAAIASGLRGKVKSNFRLKELKNMKSGLPTTKSDNFPIPLVKQKGGQYTGFEISNHNDDFIIKIPFGRWQVKKEIDKYRPWEKFDFEQVRKSPKPISLLLSTQRRKRNKGWSKDEGTEAEIRKVMNGGYQTSYIEVKRGSKTGEKSAWMLNLSIDVPKIDKGVDPSIIGGIDVGVKSPLVCAINNAFSRYSISDNDLFHFNKKMFARRRILLKKNGRKRAGHGTKNKLKPIAILTEKSGRFRKKLIERWACEIANFFIKNKVGTVQMENLESMKRKEDSYFNIRLRGFWPYAEMQNKIEFKLKQYGIKIRKVAPNNTSKTCSKCGHLNNHFSFEYRKKNKFPHFKCEKCNFKENADYNAALNISNPKLKSTKEEP

SEQ ID NO: 452 - protein, 726 aa, synthetic construct
SEVEFSHEYWMRHALTLAKRARDEREVPVGAVLVLNNRVIGEGWNRAIGLHDPTAHAEIMALRQGGLVMQNYRLSDATLYVTFEPCVMCAGAMIHSRIGRVVFGVRNSKRGAAGSLMNVLNYPGMNHCVEITEGILVDECAALLCDFYRMPRQVLSAQKRAQSSINSGGSSGGSSGSETPGTSESATPESSGGSSGGSAKNTITKALKLRIVRPYNSAEVERIVADEKNNREKIALEKNKDKVKEACSEHLKVAAYCTTQVERNACLFCKARKLDDEFYQRLRGQFPDAVFWQEISEIFRQLQKQAAEIYNQSLIELYYEIFIKGKGFANAGSVEHYLSDVCYTRAAELFKNAAIASGLRGKVKSNFRLKELKNMKSGLPTTKSDNFPIPLVKQKGGQYTGFEISSHNDDFIIKIPFGRWQVKKEIDKYRPWEKFDFEQVRKSPKPISLLLSTRRRKRNKGWSKDVGTEAEIRKVMNGDYQTSYIEVKRGSKIGEKSAWMLNLSIDVPKIDKGVDPSIIGGIDVGVKSPLVCAINSAFSRYSISDNDLFRFNKKMFARRRILLKKNRHKRAGHGAKNKLKPITILTEKSRRFRKKLIERWACEIADFFIKNKVGTVQMESLESMKRKEDSYFNTRLRGFWPYAEMQNKIEFKLKQYGIKIRKVAPNNTSKTCSKCGHLNDYFSFEYRKKNKFPHFKCEKCNFKESADYNAALNISNPKLTSSKEEP

SEQ ID NO: 453 - protein, 726 aa, synthetic construct
SEVEFSHEYWMRHALTLAKRARDEREVPVGAVLVLNNRVIGEGWNRTTGLHDPTAHAEIMALRQGGLVMRNYRLTDATLYVTFEPCVMCAGAMIHSRIGRVVFGVRNSKRGAAGSLMNVLNYPGMNHCVEITEGILVDECAALLCDFYRMPRQVLNAQKKAQSSISPGGSSGGSSGSETPGASESVTPKSSGGSSGGSAKNTITKTLKLRIVRPYNSAEVEKIVADEKNNREKIALEKNKGKVKEACSKHLKVASYCTTQVERNACPFCKARKLDDKFYQKLRGQFPDAVFWQELGEILRQLQKQAAEIYNQSLIELYYEIFIKGKGFANASSVEHYLSDVCYTRAAGLFKNAAIASGLRGKVKSNFRLKELKNMKSGLPTTKSDNFPIPLVRQKGGQYTGFEISSHNDDFIIKIPFGRWQVKKEIDKYRPWEKFDFEQVRKSPKPISLLLSTRRRKRNKGWSKDEGTEAEIRKVMNGDYQTSYIEVKRGSKIGERSAWMLNLSIDVPKIDKGVDPSIIGGIDVGVKSPLVCAINNAFSRYSIGDNDLFHYNKKMFARRRILLKKNRLKRAGHGAKNKLKPISILTEKSKRFRKKLIERWACEIADFFIKNKVGTVQIENLESMKRKEDSYFNIRLRGFWPYAEMQNKIEFKLKQYGIEIRKVAPNNTSKTCSKCGHLNSYFNFEYRKKNKFPHFKCEKCNFKENADYNAALNISNPKLKSTKEEP

SEQ ID NO: 454 - protein, 726 aa, synthetic construct
SEVEFSHEYWMRHALTLAKRARDEGEVPVGAVLVLNNRVIGEGWNRAIGLHDPTAHAEIMALRQGGLVMQNYRLIDATLYVTFEPCVMCAGAMIHSRIGRVVFGVRNNKHGAAGSLVNVLDYPGMNHRVEITEGILADECAALLCDFYRMPRQVFNARKKAQSSISPGGSSGGSSGSETPGTNESATPESSGGGFGGSAKNTITKTLQLRIVRPYNSAEVEKIVADEKNNREKIALEKNKDKVKEACSEHLKVAAYCTTRVDRNACLFCKARRLDDKFYQKLRGQFPDAVFWQEIGEIFRQLQKQAAEIYNQSLVELYYEILIKGKGIANASSVEHYLSDVCYTRAAELFKNAAIASGLRNKIKSNFRLKELRNMKSGLPTTKSDNFPIPLVKQKGGQYTGFGISNHNGDFIIKIPFGRWQVKKEINKHRPWEKFDFEQVRKSPKPISLLLSTQRRKRNKGWSKDEGTEAEIRKVMNGDYQTSYIEVKRGSKIGEKSAWMLNLSIDVPKIDKGVDPSIVGGIDVGVKSPLVCAVNNALGRYSISDNDLFHFNKKMFARRRILLKKNRHKRAGHGTKNKLKPITILTEKSGRFRKKLIERWACEIANFFIKNKVGTVQMENLESMKRKEDSYFNIRLRGFWPYAEMQNKIEFKLKQYGIKIRKVAPNNTSKTCSKCGHLNNYFSFEYRKKNKFPHFKCEKCNFKEDADYNAALNISNPKLKSTKEEP

SEQ ID NO: 455 - protein, 726 aa, synthetic construct
SEVEFSHEHWMRHALTLAKRARDEREVPVGAVLVLNNRVIGEGWNRAIGLHDPTAHAEIMALRQGGLVMQNYRLIDATLYVTFEPCVMCAGAMIHSRIGRVVFGVRNSKRGAAGSLMNVLNYPGMNHCVEITEGILVDECAALLCDFYRMPRQVLNAQKKAQSSISSGGSSGGSSGSETPGASGSVTPKSSGGSSAGSTKDTITKTLKLRIVRPYNSAEVEKVVADEKNNREKIAMEKNKGKVKEACSKHLKMASYCTTQVERNACLFCKARKLDDKFYQKLRGQFPDAVFWQELGGIFRQLQKQAAEIYNQSLIELYYEIFIKGKGITNASRVEHYLSDVCYTRAAELFKNAAIASGLRGKVKSNFRLKELKNMKSGLPTTKSDNFPIPLVKQKGGQYTGFEISSHNDDFIIKIPFGRWQVKKEIDKYRPWEKFDFEQVRKSPKPISLLLSTQRRRRNKGWGKDEGTEAEIRKVMNGDYQTSYIEVKRGSRIGEKSAWMLSLSIDVPKIDKGVDPSIIGGIDVGVKSPLVCAIGNAFSRYSISDNDLFRFNKKMFARRRILLGKNRHRRAGHGAKNKLKPITILTEKSGRFRKKLIERWACEIANFFIKNRVGTVQMENLESMKRKEDSYFNIRLRGFWPYAEMQNKIEFKLKQYGIEIRKVAPNNTSKTCSKCGHLNNYFSFEYRKKNKFPHFKCEKCNFKEDADYNAALNISNPKLKSTKEEP

SEQ ID NO: 456 - protein, 726 aa, synthetic construct
SEVEFSHEYWMRHALTLAKRARDEREVPVGAILVLNNRVIGEGWNRAIGLHDPTAHAEIMALRQGGLLMQNYRLIDATLYVTFEPCVMCAGAMIHSRIGRVVFGVRNSKHGAAGSLVNVLNYPGMNHRVEITEGVLADECAALLCDFYRMPRQVFGARKKAQSSINPGGSSGGSSGSEAPGTSESATPGSSGGSSGGSAKNTITKTLKLRIVRPYNSAEVEKIVADEKNNREKIALEKNKDKVREACSKHLKVASYCTTQVERNACPFCKARKLDDKFYQKLRGQFPDAVFWQELGEILRQLQKQAAEIYNQSLIELYYEIFIKGRGFANASSVEHYLSDVCYTRAAELFKNAAIASGLRGKVKGNFRLKELKNMKSGLPTTKSDNFPIPLVKQKGGQYTGFEISSHNDDFIIKIPFGRWQVKKEIDKYRPWEKFDFEQVRKSPKPISLLLSTQRRRRNKGWSRDEGTEAEIRKVMYGDYQTSYIEVKRGSKIGEKSTWMLNLSINVPKIDKGVDPSIIGGIDVGVKSPLVCAINNAFSRYSISDNDLFHFNKKVFARRRILLKKNRHRRAGHGAKNKLKPITILTEKSKRFRKKLIERWACEIADFFIKNKVGTVQMENLESMKRKEDSYFNIRLRGFWPYAEMQNKIEFKLKQYGIKIRKVAPNNTSRTCSECGHLNNYFSFEYRKKNKFPHFKCEKCNFKEDADYNAALNISNPKLKGTKEEL

SEQ ID NO: 457 - protein, 726 aa, synthetic construct
SEVEFSHEYWMRHALTLAKRARDEREVPVGAVLVLNNRVIGEGWNRTTGLHDPTAHAEIMALRQGGLVMRNYRLTDATLYVTFEPCVMCAGAMIHSRIGRVVFGVRNSKRGAAGSLMNVLNYPGMNHCVEITEGILVDECAALLCDFYRMPRQVLNAQKKAQSSISPGGSSGGSSGSETPGASESVTPKSSGGSSGGSAKYTITKTLKLRIVRPYNSAEVEKIVADEKNNREKIALEKNKGKVKEACSKHLEVAAYCTTQVERNACLFCKARKLDDKFYQKLRGQFPDAVFWQEIGEIFRQLQKQAAEIYNQSLIELYYEIFIKGKGLANASSVEHYLSDVCYTRAAELFKNAAIASGLRGKVKSNFRLKELKNMKSGLPTTKSDNFPIPLVKQKGGQYTGFEISSHNDDFIIKIPFGRWQVRKEIDKYRPWEKFDFEQVRKSPKPISLLLSTQRRKRNKGWSKDEGTEAEIRKVMNGDYQTSYIEVKRGSKIGEKSAWMLNLSIDVPKIDKGVDPSIIGGIDVGVKSPLVCAINNAFSRYSISDNDLFRFNKRMFARRRILLKKNRHKRAGHGAKNKLKPITILTEKSGRFRKKLIERWACEIADFFVKNKVGTVQMENLESMKRKEDSYFNIRLRGFWPYAEMQNKIEFKLKQYGIKVRKVAPNNTSKTCSKCGHLNNYFSFEYRKKNKFPHFKCEKCNFKENADYNAALNISNPKLKSTKEEP

SEQ ID NO: 458 - protein, 726 aa, synthetic construct
SEVEFSHEYWMHHALTLAKRARDEREVPVGAVLVLNNRVIGEGWNRAIGLHDPTAHAEIMALRQGGLVMQDYRLSDATLYVTFEPCVMCAGAMIHSRIGRVVFGVRNSKRGAAGSLMNVLNYPGMNHCVEITEGILVDECAALLCDFYRMPRQVLSAQKKAQSSISSGGSSGGSSGSETPGASGSVTPKSSVGSSAGSTKNTITKTLKLRIVRPYNSAVVEKIVADEKNNREKIALEKNKDKVKEACSKHLKVAAYCTTQVERNACLFCKARKLDDKFYQKLRGQFPDAVFWQELGGIFRQLQKQAAEIYNQSLIELYYEIFIKGKGITNASRVEHYLSDVCYTRAAELFKNAAIASGLRGKVKSNFRLKELKNMKSGLPTTKSDNFPIPLVKQKGGQYTGFEISSHNDDFIIKIPFGRWQVKKEIDKYRPWEKFDFEQVRKSPKPISLLLSTQRRKRNKGWSKDEGTEAEIRKVMNGDYQTSYIEVKRGSRIGEKSAWMLSLSIDVPKIDRGVDPSIIGGIDVGVKSPLVCAINNALSRYSISDNDLFHFNKKMFARRRILLKKNRHRRAGHGARNKLKPITVLTEKSKRFRKKLIERWACEIANFFIKNKVGTVQMENLESMRRKEDSYFNIRLRGFWPYAEMQNKIEFKLKQYGIEIRKVAPNNTSKTCSKCGHLNSYFNFEYRKKNKFPHFKCEKCNFKENADYNAALNISDPKLRSTKEEP

SEQ ID NO: 459 - protein, 726 aa, synthetic construct
SEVEFSHEYWMRHALTLAKRARDEREVPVGAVLVLNNRVIGEGWNRAIGLHDPTAHAEIMALRQGGLVMQNYRLTDATLYVTFEPCVMCAGAMIHSRIGRVVFGVRNSKRGAAGSLMNVLNYPDMNHCVEITEGILVDECAALLCDFYRMPRQVLNAQKKAQSSISSGGSSGGSSGSVTPGTSGSATPEGSGGSSSGFAKNTITKTLKLRIVRPYNSAEVEKIVVDEKNNREKVALEKNKDKVKEACSEHLKVAAYCTTQVERSACLFCKARKLDDKFYQKLRGQFPDAVFWQEIGEIFRQLQKQAAEIYNQSLIELYYEIFIKGKGFANASSVEHYLSDVCYTRAAELFKNAAIASGLRGKVKSNFRLKELKNMKSGLPTTKSDNFPIPLVKQKGGQYTGFEISSHNDDFIIKIPFGRWQVKKEIDKYRPWEKFDFEQVRKSPKPISLLLSTQRRKRNKGWSKDEGTEAEIRKVMNGDYQTSYIEVKRGSKTGEKSAWMLNLSIDVPKIDKGVDPSIIGGIDVGVKSPLVCAINNAFSRYSISDNDLFRFNKKMFARRRILLRKNRHKRAGHGAKNKLKPISILTEKSGRFRKKLIERWACEIADFFIKNKVGTVQMENLEGMKRKEDSYFNIRLRGFWPYAEMQNKIEFKLKQYGIEIRKVAPNNTSKTCSKCGHLNNYFNFEYRKKNKFPHFKCEKCNFKENADYNAALNISNPKLKSTKEEP

SEQ ID NO: 460 - protein, 726 aa, synthetic construct
SEVEFSHEYWMRHALTLAKRARDEREVPVGAVLVLNNRVIGEGWNRAIGLHDPTAHAEIMALRQGGLVLQNYRLVDATLYVTFEPCVLCAGAMVHSRIGRVVFGARNSKRGAAGSLMNILNYPGMNHRVEITEGILADECAALLCDFYRMPRQVFNAQKKAQSSINSGGSSGGSSGSETPSTSESATPESSGGSSGGSAKNTITKTLQLRIVRPYNSAEVEKIVTDEKNNREKIALEKNKDKVKEACSKHLKMASYCTTQVERNACLFCKARKLDDKFYQKLRGQFPDAVFWQELGGIFRQLQKQAAEIYNQSLIELYYEIFIKGKGITNASRVEHYLSDVCYTRAAELFKNAAIASGLRSKVRSNFRLKELKNMKSGLPTTKSDNFPIPLVKQKGGQYTGFEISSHNDDFIIKIPFGRWQMKKEIDRYRPWEKFDFEQVRKSPKPISLLLSTQRRKRNKGWSKDEGTEAEIRKVMNGDYQTSYIEVKRGSKIGEKSAWMLNLSIDVPKIDKGVDPSIIGGIDVGVKSPLVCAINDAFSRYSISDNDLFHFNKKMFARRRILLKKSKHKRAGHGAKNKLKPITILTEKSRRFRKKLIERWACEIADFFIKNKVGTVLMENLESMKRREDSYFNIRLRGFWPYAEMQNKIEFKLKQYGIEVRKVAPNNTSKTCSKCGHLNNYFNFEYRKKNKFPLFKCEKCNFKENADYNAALNISNPKLKSTKEEP

SEQ ID NO: 461 - protein, 726 aa, synthetic construct
SEVEFSHEYWMRHALTLAKRARDEREVPVGAVLVLNNRVIGEGWNRAIGLHDPTAHAEIMALRQGGLVMQNYRLTDATLYVTFEPCVMCAGAMIHSRIGRVVFGVRNSKRGAAGSLMNVLNYPGMNHCVEITEGILVDECAALLCDFYRMPRQVLSAQKKAQSSIGPGGSSGGSSGSETPGASGSVTPKSSGGSSAGSTKDTITKTLKLRIVRPYNSAEVEKIVADEKNSREKIALEKNKDKVKEACSEHLKVAAYCTTQVERNACLFCKARKLDDRFYQKLRGQFPDAVFWQEIGEIFRQLQKQAAEIYNQSLVELYYEILIKGKGFANASSVEHYLSDVCYTRAAELFKNAAIASGLRGKVKSNFRLKELKNMKSGLPTTKSDNFPIPLVKQKGGQYTGFEISSHNDDLIVKIPFGRWQVKKEIDRYRPWEKFDFEQVRKSPKPISLLLSTQRRKRNKGWSKDEGTEAEIRKVMNGDYQTSYIEVRRGSKIGEKNAWMLSLSIDVPKIDKGADPSIIGGIDVGVKSPLVCAINNAFSRYSISDNDLFRFNKKMFARRRILLKKNRHKRAGHGAKNKLKPISILTGKSERFRKKLIERWACEIADFFIKNKVGTVQMENLESMKRKEDSYFNIRLRGFWPYAEMQNKIEFKLKQYGIEIRKVAPNNTSKTCSKCGHLNNYFNFEYRKKNKFPHFKCEKCNFKENADYNAALNISNPKLKSTKEEP

SEQ ID NO: 462 - protein, 726 aa, synthetic construct
SEVEFSHEYWMRHALALAKRARDEREVPVGAVLVLNNRAIGEGWNRAIGLHDPTAHAEIMALRQGGLVMQNYRLTDATLYVTFEPCVMCAGAMIHSRIGRVVFGVRNSKRGAAGSLMNVLNYPGMNHCVEITEGILVDECAALLCDFYRMPRQVLNAQKKAQSSISSGGSSGGSSGSETPGASGSVTPKSSGGSSAGSTKDTITKTLKLRIVRPYNSAEVEKVVADEKNNREKIAIEKYKDMVKEACSKHLKVASYCTTQVERNACLFCKARKLDDKFYQKLRGQFPDAVFWQELGGIFRQLQKQAAEIYNQSLIELYYEIFIKGKGITNASRVEHYLSDVCYTRAAELFKNAAIASGLRSKVRSNFRLKELKNMKSGLPTTKSDNFPIPLVKQKGGQYTGFEISSHNSDFIIKIPFGRWQEKEEIGKYRPWEKFDFEQVRRSPKPISLLLSTQRRKKNKGWSKDEGTEAEIRRVMNGDYQTSYIEVKRGSKIGEKSAWMLNLSIDVPKIDKGVDPSIIGGIDVGVKSPLVCAINNAFSRYSISDNDLFHFNKKMFARRRILLKRNRRRRAGHGAKNKLKPITILTEKSVRFRKKLIERWACEIADFFIKNKVGTVQMENLESMKRKEDSYFNIRLRGFWPYAEMQNKIEFKLKQYGIEIRRVAPNNTSRTCSKCGHLNNYFNFEYRRKYKFPHFKCEKCNFKEDADYNAALNISNPKLKSTKEEP

SEQ ID NO: 463 - protein, 726 aa, synthetic construct
SEVEFSHEYWMRHALTLAKRARDEREVPVGAILVLNNRVIGEGWNRAIGLHDPTAHAEIMALRQGGLVMQNYRLIDATLYVTFEPCVMCAGAMIHSRIGRVVFGVRNNKHGAAGSLVNVLNYPGMNHRVEITEGILADECAALLCDFYRMPCQVFNARRKAQSSIDSGGSSDGSGGSVTPGTSGSATPEGSGGSSSGFAKNTITKTLKLRIVRPYNSAEVEKIVADEKNNREKIALEKNKDKVKEACSKHLKVATYCTTQVERNACLFCKARKLDDKFYRKLRGQFPDAVFWQELGEIFRQLQKQAAEIYNQSLIELYYEIFIKGKGFANASSVEHYLSDVCYTRAAELFKNAAIASGLRGKVKSNFRLKELKNMKSGLPTTKSDNFPIPLVKQKGGQYTGFEISSHNDDFIIKIPFGRWQVKKEIDKYRPWEKFDFEQVRKSPKPISLLLSTQRRKRNKGWSKDEGTEAEIRKVMNGDYQTSYIEVKRGSKTGEKSAWMLNLSIDVPKIDKGVDPSIIGGIDVGVKSPLVCAINNAFSRYSISDNDLFRFNKKMFARRRILLGKNRHKRAGHGVKNKLKPITILTEKSGRFRKKLIERWACEIANFFIKNKVGTVQMENLESMKRKEDSYFNIRLRGFWPYAEMQNKIEFKLKQYGIVVRKVAPNNTSKTCSKCGHLNNYFNFEYRKKNKFPHFKCEKCNFKEDADYNAALNISNPKLKGTKEEL

SEQ ID NO: 464 - protein, 726 aa, synthetic construct
SEVEFSHEYWMRHALTLAKRARDEREVPVGAVLVLNNRVIGEGWNRTIGLHDPTAHAEIMALRQGGLVMQNYRLTDATLYVTFEPCVMCAGAMIHSRIGRVVFGVRNSKRGAAGSLMNVLNYPGMNHCVEITEGILVDECAALLCDFYRMPRQVLNAQKKAQSSISSGGSSGGSSGSETPGASESVTPKSSVGSSAGSAKNTITKTLQLRIVRPYNSAEVEKIVADEKNNREKIALEKNKDKVKEACSKHLKVASYCTTQVERNACPFCKARKLDDKFYQKLRGQFPDAVFWQELGEIFRQLQKQAAEIYNQSLIELYYEIFIKGKGFANASSVEHYLSDVCYTRAAELFKNAAIASGLRGKVKSNFRLKELKNMKSGLPTTKSDNFPIPLVKQKGGQYTGFEISSHNDDFIIKIPFGRWQVKKEINKYRPWEKFDFEQVRKSPKPISLLLSTQRRKRNKGWSKDEGTEAEIRKVMNGDYQTSYIEVKRGSKIGEKSAWMLNLSIDVPKIDKGVDPSIIGGIDVGVKSPLVCAISNAFSRYSISDNDLFHFNKKMFARRRILLKKSKHKRAGHGAKNKLKPITILTEKSRRFRKKLIERWACEIADFFIKNKVGTVQMENLESMKRKEDSYFNIRLRGFWPYAEMQNKIEFKLKQYGIEIRKVAPNNTSKTCSRCGHLNNYFNFEYRRKNKFPHFKCEKCNFKENADYNAALNISNPKLKSTKEEP

SEQ ID NO: 465 - protein, 726 aa, synthetic construct
SEVEFSHEYWMRHALTLAKRARDEREVPVGAVLVLNNRVIGEGWNRAIGLHDPTAHAEIMALRQGGLVMQNYRLTDATLYVTFEPCVMCAGAMIHSRIGRVVFGVRNSKRGAAGSLMNVLNYPGMNHCVEITEGILMDECAALLCDFYRMPRQVLNAQKKAQSSISSGGPSGGSSCSETPGASESVTPKSSGGSSTGSTKNTITKTLKLRIVRPYNSAEVEKIVADEKNSREKIALEKNKDKVKEACSEHLKVAAYCTTQVERNACLFCKARKLDDRFYQKLRGQFPDAVFWQEIGEIFRQLQKQAAEIYNQSLVELYYEIFIKGKGIANASSVEHYLSDVCYTRAAELFKNAAIASGLRNKIKSNFRLKELRNMKSGLPTTKSDNFPIPLVRQKGGQYTGFEISNHNGDFIIKIPFGRWQVKKEICKHRPWEKFDFEQVRKSPKPISLLLGTQRRKRNKGWGKDEGTEAEIRKVMNGDYQTSYIEVKRGSKIGEKSAWMLNLSIDVPKIDKGVDPSIIGGIDVGVKSPLVCAINNALSRYSISDNDLFHFNKKMFARRRILLRKNRHKRAGHGARNKLKPITVLTEKSERFRKKLIERWACEIANFFIKNKVGTVQMENLESMKRREDSYFNVRLRGFWPYAEMQSKIEFKLKQYGIKIRKVAPNNTSKTCSKCGHLNNYFNFEFRKKNKFPHFKCEKCNFKEDADYNAALNISNPKLKSTKEEP

SEQ ID NO: 466 - protein, 726 aa, synthetic construct
SEVEFSHEYWMRHALTLAKRARDEREVPVGAVLVLNNRVIGEGWNRAIGLHDPTAHAEILALRQGGLVMQNYRLTDATLYVTFEPCVMCAGAMIHSRIGRVVFGVRNSKRGAAGSLMNVLNYPGMNHCVEITEGILMDECAALLCDFYRMPRQVLNAQKKAQSSISSGGPSGSSSCSETPGASESVTPKSSGGSSIGSTKNTITKTLKLRIVRPYNSAEVEKIVADEKNSREKIALEKNKDKVKEACSEHLKVAAYCTTQVERNACLFCKARKLDDRFYQKLRGQFPDAVFWQEIGEIFRQLQKQAAEIYNQSLIELYYEIFIKGKGFAIASSVEHYLSCVCYTRAAELFKNAAIASGLRGKVKSNFRLKELKNMKSGLPTTKSDNFPIPLVKQKGGQYTGFEISSHNDDFIIKIPFGRWQVKKEIDKYRPWEKFDFEQVRKSPKPISLLLSTQRRKRNKGWSKDEGTEAEIRKVMNGDYQTSYIEVKRGSKIGEKSAWMLSLSIDVPKIDKGVDPSIIGGIDVGVRSPLVCAINNALCRYSISDNDLFHFNKKMFARRRILLKKSRHKRAGHGAKNKLKPISILTEKSKRFRKKLIERWACEIADFFIKNKVGTVQMENLESMKRKEDSYFNIRLRGFWPYAEMQNKIEFKLKQYGIEIRKVAPNNTSKTCSKCGHLNNYFNFEYRKKNKFPHFKCEKCNFKENADYNAALNISNPMLKSTKEEP

SEQ ID NO: 467 - protein, 726 aa, synthetic construct
SEAEFSHEYWMRHALTLAKRARDEREVPVGAVLVLNNRVIGEGWNRAIGLHDPTAHAEIMALRQGGLVMQNYRLTDATLYVTFEPCVMCAGAMIHSRIGRVVFGVRNSKRGAAGSLMNVLNYPGMNHCVEITEGILVDECAALLCDFYRMPRQVLSAQKKAQSSISPGGSSGGSSGSETPGASGSVTPKSSGGSSAGSTKDTITKTLKLRIVRPYNSAEVEKIVADEKNSREKIALEKNKDKVKEACSEHLKVAAYCTTQVERNACLFCKARKLDDRFYQKLRGQFPDAVFWQEIGEIFRQLQKQAAEIYNQSLIELYYEIFIKGKGFANASSVEHYLSDVCYTRAAELFKNAAIASGLRGKVKSNFRLKELKNMKSGLPTTKSDNFPIPLVKQKGGQYTGFEISNHDSDFIIKIPFGRWQAKKEIDKYRPWEKFDFEQVRKSPKPISLLLSTQRRKKNRGWSKDEGTEAEIKKVMNGDYQTSYIEVKRGSKIGEKSAWMLNLSIDVPKIDKGVDPSIIGGIDVGVKSPLVCAISNAFSRYSISDNDLFHFNKKMFARRRILLKKSKHKRAGHGAKNKLKPITILTEKSRRFRKKLIERWACEIADFFIKNKVGTVQMENLESMKRREDSYFNIRLRGFWPYAEMQNKIEFKLKQYGIEIRKVAPNNTSKTCSKCGHLNNYFNFEYRKKNKFPHFKCEKCNFKENADYNAALNISNPKLKSTKEEP

SEQ ID NO: 468 - protein, 726 aa, synthetic construct
SEVEFSHEYWMRHALTLAKRARDEREVPVGAVLVLNNRVIGEGWNRAIGLHDPTAHAEIMALRQGGLVMQNYRLTDATLYVTFEPCVMCAGAMIHSRIGRVVFGVRNSKRGAAGSLMNVLNYPGMNHCVEITEGILMDECAALLCDFYRMPRQVLSAQKKAQSSISSGGPSGGSSCSETPGASESVTPKSSGGSSGGSAKNTITKTLKLRIVRPYNSAEVEKIVADEKNNREKIALEKNKGKVKEACSKHLGVAAYCTTQVERNACLFCKARKLDDKFYQKLRGQFPDAVFWQELGEIFRQLQKQAAEIYNQSLIELYYEIFIKGKGIANASSVEHYLSDVCYTRAAELFKNAAIASGLRGKVKSNFRLKELKNMKSGLPTTKSDNFPIPLVKQKGGQYTGFEISSHNDDFIIKIPFGRWQVKKEINKHRPWEKFDFEQVRKSPKPISLLLSTQRRKRNKGWSKDEGTEAEIRRAMNGDYQTSYIEVKRGSKIGEKSAWMLSLSIDVPKIDKGVDPSIIGGIDVGVKSPLVCAINNAFCRYSISDNDLFHFNKKMFARRRILLKKSRHKRAGHGAKNKLKPISILTEKSKRFRKKLIERWACEIADFFIKNKVGTVQMENLESMKRKEDSYFNIRLRGFWPYAEMQNKIEFKLKQYGIEIRKVAPNNTSKTCSKCGHLNNYFNFEYRKKNKFPHFKCEKCNFKENADYNAALNISNPKLKSTKEEP

SEQ ID NO: 469 - protein, 726 aa, synthetic construct
SEVEFSHEYWMRHALTLAKRARDEREVPVGAVLVLNNRVIGEGWNRAIGLHDPTAHAEIMALRQGGLVMQNYRLTDATLYVTFEPCVMCAGAMVHSRIGRVVFGVRNSKRGAAGSLMNVLNYPGVNHCVEITEGILVDECAALLCDFYRMPRQVLNAQKKAQSSISSGGSSGGCSGSEMPGASESVTPKSSGGSSAGSTKNTITKTLKLRIVRPYNSAEVEKIVADEKNSREKIALEKNKDKVKEACSEHLKVAAYCTTQVERNACLFCKARKLDDRFYQKLRGQFPDAVFWQETGEIFRQLQKQAAEIYNQSLIELYYEIFIKGKGFANASSVEHYLSDVCYTRAAELFKNAAIASGLRGKVKSNFRLKELKNMKSGLPTTKSDNFPIPLVKQKGGQYTGFEISSHNDDFIIKIPFGRWQVKKEIDKYRPWEKFDFEQVRKSPKPISLLLSTQRRKRNKGWSKDEGTEAEIRKVMNGDYQTSYIEVKRGSKIGEKSAWMLNLSIDVPKIDKGVDPSIIGGIDVGVKSPLVCAINNAFSRYSISDNDLFRFNKKVFARRRILLRKNRHKRAGHGAKNKLKPITIMTEKSKRFRKKLIERWACEIADFFIKNKVGTVQMENLESMKRKEDSYFNIRLRGFWPYAEMQNKIEFKLKQYGIVVRKVAPNNTSKTCSQCGHLNNYFNFEYRKKNKFPYFKCEKCNFKENADYNAALNISNPQLKSTKGEP

SEQ ID NO: 470 - protein, 726 aa, synthetic construct
SEVEFSHEYWMRHALSLAKRARDEREVPVGAVLVLNNRIIGEGWNRAIGQHDPTAHAEIMALRQGGLVMQNYRLTDATLYVTFEPCVMCAGAMVHSRIGRVVFGVRNSKRGAAGSLMNVLNYPGVNHCVEITEGILVDECAALLCDFYRMPRQVLNAQKKAQSSISSGGSSGGCSGSEMPGASESVTPKSSGGSSAGSTKNTITKTLKLRIVRPYNSAEVEKIVADEKNSREKIALERNKDKVKEACSEHLKVAAYCTTQVERNACLFCKARKLDDRFYQKLRGQFPDAVFWQEAGEIFRQLQRQAAEIYNQSLIELYYEIFIKGKGFANASSVEHYLSDVCYTRAAELFKNAAIASGLRGKVKSNFRLKELKNMKSGLPTTKSDNFPIPLVKQKGGQYTGFEISSHNDDFIIKIPFGRWQMKKEIDRYRPWEKFDFEQVRKSPKPISLLLSTQRRKRNKGWSKDEGTEAEIRRVMNGDYQTSYIEVKRGSKIGEKSAWVLSLSIDVPKIDKGVDPSIIGGIDVGVRSPLVCAISNALSRYSINDNDLFHFNKKMFARRRILLKKSKHKRAGHGAKNKLKPITILTEKSRRFRKKLIERWACEIADFFIKNKVGTVQMENLEGMKRKEDSYFNIRLRGFWPYAEMQDKIEFKLKQYGIKVRKVAPNNTSKTCSKCGHLNNYFNFEYRKKNRFPHFKCEKCNFKEDADYNAALNISNPKLKSTKGEP

SEQ ID NO: 471 - protein, 726 aa, synthetic construct
SEVEFSHEYWMRHALTLAKRARDEREVPVGAVLVLNNRVIGEGWNRAIGLHDPTAHAEIMALRQGGLVMQNYRLTDATLYVTFEPCVMCAGAMIHSRIGRVVFGVRNSKRGAAGSLMNVLNYPGMNHCVEITEGILMDECAALLCDFYRMPRQVLNAQKKAQSSISSGGPSGGSSGSEAPGTSESATPKSSGGSSGGSAKNTITKALKLRIVRPYNSAEVEKIVADEKNNRERIALEKNKDKVKEACSKHLKVAAYCTTQVERNACLFCKARKLDDKFYQKLRGQFPDAVFWQELGEIFRQLQKQAAEIYNQSLIELYYEIFIKGKGFANASSVEHYLSDVCYTRAAELFKNAAIASGLRGKVKSNFRLKELKNMKSGLPTTKSDNFPIPLVKQKGGKYTGFEISSHNDDFIIKIPFGRWQVKKEIDKYRPWEKFDFEQVRKSPKPISLLLSTQRRKRNKGWSKDEGTEAEIRKVMNGDYQTSYIEVKRGCKIGEKSAWMLNLSIDVPKIDKGVDPSIIGGIDVGVKSPLVCAINNAFSRYSISDNDLFHFNKKMFARRRILLKKNRHKRAGHGAKNKLKPISILTEKSKRFRKKLIERWACEIANFFIKNKVGTVQMEDLESMKRREDSYFNIRLRGFWPYAEMQSKIEFKLKQYGIKIRKVAPNNTSKTCSKCGHLNNYFNFEYRKKNKFPHFKCEKCNFKEDADYNAALNISNPKLKSTKEEP

SEQ ID NO: 472 - protein, 726 aa, synthetic construct
SEVEFSHEYWMRRALTLAERARDEREVPVGAVLVLNSRVIGVGWNRAIGLHDPTAHAEIMALRQGGLVMRNHRLIDATLYVTFEPCVMCAGAMVHSRIGRVVFGVRNNKHGAAGSLVNVLNYPGMNHRVEITEGILADECAALLCDFYRMPRQVFNARKKAQSSINPGGSSGGSSGSETPGTSESPTPESSGGSSAGSTKNTITKTLKLRIVRPYNSAEVEKIVADEKNSREKIALEKNKDKVKEACSEHLKVAAYCTTQVERNACLFCKARKLDDKFYQKLRGQFSDAVFWQEIGEIFRQLQKQAAEIYNQSLIELYYEILIKGKGFANASSVEHYLSDVCYTRAAELFKNAAIASGLRGKVKSNFRLKELKNMKSGLPTTKSDNFPIPLVKQKGGKYTGFEISSHNDDFIIKIPFGRWQVKKEIDKYRPWEKFDFEQVRKSPKPISLLLSTQRRKRNKGWSKDEGTEAEIRKVMKGDYQTSYIEVKRGSKIGEKSAWMLNLSIDVPKIDKGVDPSIIGGIDVGVKSPLVCAINNAFGRYSISDNDLFHFNKKMFARRRILLKKNRHRRAGHGAKNKLKPITILTEKSKRFRKKLIERWASEIADFFIKNKVGTVQMENLESMKRREDSYFNIRLRGFWPYAEMQNKIEFKLKQYGVEIRKVAPNNTSKTCSKCGHLNNYFNFEYRKKNKFPHFKCEKCNFKENADYNAALNISNPKLKSTKEEH

SEQ ID NO: 473 - protein, 726 aa, synthetic construct
SDVEFSHEYWMRHALTLAKRARDEREVPVGAVLVLNNRVIGEGWNRAIGLHDPTAHAEIMALRQGGLVMQNHRLVDATLYVTFEPCVMCAGAMIHSRIGRVVFGVRNSKRGAAGSLMNVLNYPGMNHCVEITEGILVDECAALLCDFYRMPRQVLNAQKKAQSSISSGGSSGGSSGSETSGTSGSATPEGSGGSSDGSAKNTITKTLKLRIVRPYNSAEVEKIVADEKNNREKIALEKNKDKVKEACSKHLKVASYCTTQVERNACLFCKARKLDDKFYQKLRGQFPDAVFWQELGEIFRQLQKQAAEIYNQSLIELYYEIFIKGKGFANASSVEHYLSDVCYTRAAELFKNAAIASGLRGKVKSNFRLRELKNMKSGLPTTKSDNFPIPLVKQKGGQYTGFEISSHNDDFIIKIPFGRWQVKEEIDKYRPWEKFDFEQVRKNPKPISLLLSTQRRKRNKGWSKDEGTEAEIKKVMSGDYRTSYIEVKRGSKIGEKSAWMLSLSIDVPKIDRGVDPSIIGGIDVGVKSPLVCAINNAFSRYSISDNDLFRFNKKMFARRRILLKKNRHKRAGHGAKNKLKPISILTGKSERFRKKLIERWACEIADFFIKNKVGTVQMENLESMKRKEDSYFNIRLRGFWPYAEMQNKIEFKLKQYGIEIRKVAPNNTSKTCSKCGHLNNYFNFEYRKKNKFPHFKCEKCDFKENADYNAALNISNPKLKSAKKEP

SEQ ID NO: 474 - protein, 726 aa, synthetic construct
GEVEFSHEYWMRHALTLAKRARDEREVPVGAVLVLNNRVIGEGWNRAIGLHDPTAHAEIMALRQGGLVMQNYRLIDATLYVTFEPCVMCAGAMIHSRIGRVVFGVRNSKHGAAGSLVNVLNYPGMNHRVEITEGILADECAALLCDFYRMPRQVFNARKKAQSSINPSGSSGGSSGSVTPGTSESATPESSGGGFGGSAKNTITKTLQLRIVRPYNSAEVEKIVADEKNNREKIALEKNKDKVKEACSKHLKMASYCTTQVERNACLFCKARKLDDKFYQKLRGQFPNAVFWQELGGIFRQLQKQAAEIYNQSLIELYYEIFIKGKGITNASRVEHYLSDVCYTRAAELFKNAAIASGLRSKVRSNFRLKELKNMKSGLPTTKSDNFPIPLVKQKGGQYTGFEISSHNSDFIIKIPFGRWQVKEEIDKFRPWEKFDFGQVRKSPKPISLLLSTQRRKKNKGWSKDEGTEAEIRRVMNGDYQTSYIEVKRGSKIGEKSAWMLNLSIDVPKIDKGVDPSIIGGIDVGVKSPLVCAINNSSSRYSICDNDLFRFNKKMFARRRILLKKNRHKRAGHGAKNKLKPITILTEKSGRFRKKLIERWACEIADFFIKNKVGTVQMENLEGMKRKEDSYFNIRLRGFWPYAEMQNKIEFKLKQYGIEIRKVAPNNTSKTCSKCGHLNNYFNFEYRKKNKFPHFKCEKCNFKENADYNAALNISNPRLKSTKEEP

SEQ ID NO: 475 - protein, 726 aa, synthetic construct
SEVEFSHEYWMRHALTLAKRARDEREVPVGAVLVLNNRVIGEGWNRAIGLHDPTAHAEIMALRQGGLVMQNYRLVDATLYVTFEPCVMCAGAMIHSRIGRVVFGVRNNKHGAAGSLMNVLNYPGMNHRVEITEGILADECAALLCDFYRMPRQVFNARKKAQSSINPGGPSGGSSGSKTPGTSESATPEGSGGSSGGSAKNTITKTLKLRIVRPYNSAEVEKIVADEKNNREKIALEKNKGRVKEACSKHLKMASYCTTQVERNACLFCKARKLDDKFYQKLRGQFPDAVFWQELGGIFRQLQKQAAEIYNQSLIELYYEIFIKGKGITNASRVEHYLSDVCYTRAAELFKNAAIASGLRSKVRSNFRLKELKNMKSGLPTTKSDNFPIPLVKQKGGQYTGFEISSHNSDFIIKIPFGRWQVKEEIDKYRPWEKFDFEQVRKSPKPISLLLSTQRRKKNKGWSKDEGTEAEIRRVMNGDYQTSYIEVRRGSKIGEKSAWMLSLSIDVPKIDKGVDPSIIGGIDVGVKSPLVCAINNSFSRYSICDNDLFRFNKKMFARRRILLKNNRHKRAGHGAKNKLKPITILTKKSERFRKKLIERWACEIADFFIKNKVGTVQMENLESMKRKEDSYFNIRLRGFWPYAEMQNKIEFKLKQYGIEIRKVAPNYTSKTCSKCGHLNNYFNFEYRKKNKFPHFKCEECNFKENADYNAALNISNPKLKSTKEKP

SEQ ID NO: 476 - protein, 726 aa, synthetic construct
SEVEFSHEYWMRHALTLAKRARDEREVPVGAVLVLNNRVIGEGWNRAIGLHDPTAHAEIMALRQGGLVMQNYRLIDATLYVTFEPCVMCAGAMVHSRIGRVVFGVRNSKRGAAGSLMNVLDYPGMGHRVEITEGILANECAALLCDFYRMPRQVFNARKKAQSSINPSGSSGGSSGSVTPGTSESATPESSSGGFGGSAKNTITKTLQLRIVRPYNSAEVEKIVADEKNNREKIALEKNKDKVKEACSKHLKVASYCTTQVERNACLFCKARKLDDKFYQKLRGQFPDAVFWQELGEIFRQLQKQAAEIYNQSLIELYYVIFIKGKGLANASSVEHYLSDVCYTRAAELFKNAAIASGLRGKVKSNFKLKELKSMKSGLPSTKSDNFPIPLVKQKGGQYTGFEISSHNDDFIIKIPFGRWQVKKEIDKYRPWEKFDFEQVRKSPKPISLLLSTQRRKRNRGWSKDEGTEAEIRKVMNGDYQTSYIEVKRGSKIGEKSAWMLNLSIDVPKIDKGVDPSIIGGIDVGVKSPLVCAINNAFSRYSISDNDLFRFNKKMFARRRILLGKNRHKRAGHGVKNKLKPITILTEKSGRFRKKLIERWACEIADFFVKNKVGTVQMENLESMKRKEDSYFNIRLRGFWPYAEMQNKIEFKLKQYGIKVRKVAPNNTSKTCSKCGHLNNYFSFEYRKKNKFPHFKCEKCNFKENADYNAALNISNPKLKSTKEEP

SEQ ID NO: 477 - protein, 726 aa, synthetic construct
SEVEFSHEYWMRRALTLAKRARDEREVPVGAVLVLNNRVIGVGWNRAVGLHDPTAHAEIMALRQGGLVMQNYRLIEATLYVTFEPCIMCAGAMIHSRIGRVVFGVRNNKRGAAGSLMNVLNYPGMNHRVEITEGILADECAALLCDFYRMPRQVFNARKKAQSSINSGGSSGGSSGSETPGTSESATPKSSGGSSGGSAKNTITKTLKLRIVRPYNSTEVERIVADEKNNREKIALEKNKDKVKEACSKHLKAASYCTTQVERNACLFCKARKLDDKFYQKLRGQFPDAVFWQEIGEIFRQLQKQAAEIYNQSLIELYYEIFIKGKGLANASSVEHYLSDVCYTRAAELFKNAAIASGLRGKVKSNFRLKELKNMKSGLPTTKSDNFPIPLVKQKGGQYTGFEISSHNDDFIIKIPFGRWQVKEEIDKFRPWEKFDFEQVRKSPKPISLLLSTQRRKKNKGWSKDEGTEAEIRRVMNGDYQTSYIEVKRGSKIGEKSAWMLNLSIDVPKIDKGVDPSIIGGIDVGVKSPLVCAINNAFSRYSISDNDLFRFNKKMFARRRILLKKNRHKRAGHGAKNKLKPISILTGKGERFRKKLIERWACEIADFFIKNKVGTVQMENLESMKRKEDSYFNIRLRGFWPYAEMQNKIEFKLKQYGIEVRKVAPNNTSKTCSKCGHLNNYFNFEYRKKNKFPHFKCEKCNFKENADYNAALNISNPKLKGTKEEP

SEQ ID NO: 478 - protein, 726 aa, synthetic construct
SEVEFSHEHWMRHALTLAKRARDEREVPVGAVLVLNNRVIGEGWNRAIGLHDPTAHAEIMALRQGGLVMQNHRLIDATLYVTFEPCVMCAGAMIHSRIGRVVFGVRNNKRGAAGSLMNVLNYPGMNHRVEITEGILAGECAALLCDFYRMPRQVLNAQKRARSCINSGGSSGGSSGSDTPGTSESATPESSGGSSGGSAKNTITKTLKLRIVRPYNSAEVEKIVADEKDNREKIALEKNKGKVKEACSKHLKVAAYCTTQVERNACLFCKARRLDDKFYQKLRGQFPDAVFWQEIGEIFRQLQKQAAEIYNQSLIELYYEIFIKGKGFANASSVEHYLSDVCYTRAAELFKNAAIASGLRGKVKSNFRLKELKNMKSGLPTTKSDNFPIPLVKQKGGQYTGFEISSHNDDFVIKIPFGRWQVKKEIDKYRPWEKFDFEQVRKSPKPISLLLSTQRRKRNKGWSKDEGTEAEIRKVMNGDYQTSYIEVKRGSKIGEKSAWMLNLSIDVPRIDKGVDPSIIGGIDVGVKSPLVCAINNALSRYSISDNDLFHFNKKMFARRRILLKKNRHRRAGHGARNKLKPITVLTEKSKRFRKKLIERWACEIANFFIKNKVGTVQMENLESMKRKEDSYFNIRLRGLWPYAEMQNKIEFKLKQYGIEVRKVAPNNTSKTCSKCGHLNNYFNFEYRKRNKFPHFKCEKCNFKENADYNAALNISNPKLKGTKEEP

SEQ ID NO: 479 - protein, 726 aa, synthetic construct
SEAEFSHEYWMRHALTLAKRARDEREVPVGAVLVLNNRVIGEGWNRAIGLHDPTAHAEIMALRQGGLVMQNYRLADATLYVTFEPCVLCAGAMVHSRIGRVVFGVRNNKRGAAGSLMNILNYPGMNHRVEITEGILADECAALLCDFYRMPHQVFNAQKKAQSSINSGGSSGGSSGSVTPGPSESATPESSGGSSAGSTKDAITKTLKLRIVRPYNSAEVEKIVADEKNNREKIALEKNKDKVKEACSEHLKVAAYCTTQVERSACLFCKARKLDDKFYQKLRGRFPDAVFWQEIGEIFRQLQKQAAEIYNQSLIELYYEIFIKGKGFANASSVEHYLSDVCYTRAAELFKNAAIASGLRGKVKSNFRLKELRNMKSGLPTTKSDNFPIPLVKQKGGQYTGFEISSHNDDFIIKIPFGRWQVKKEIDKYRPWERFDFEQVRKSPKPISLLLSTQRRKRNKGWSKDEGTEAEIRKVMNGDYQTSYIEVKRGSKIGEKSAWMLNLSIDVPKIDKGVDPSIIGGIDVGVKSPLVCAINNALSRYSISDNDLFHFNKKMFARRRILLRKNRHKRAGHGAKNKLKPITMMTEKSKRFRKKLIERWACEIADFFIKNKVGTVQMENLESMKRKEDSYFNIRLRGFWPYAEMQDKIEFKLKQYGIVVRKVAPNNTSKTCSKCGHLNHYFNFEYRKKNKFPHFKCEKCNFKEDADYNAALNISNPKLKSTKGEP

SEQ ID NO: 480 - protein, 726 aa, synthetic construct
SGVEFSHEYWMRHALTLAKRARDEREVPVGAVLVLNNRVIGVGWNRAVGLHDPTAHAEIMALRQGGLVMQNYRLVDATLYVTFEPCVMCAGAMIHSRIGRVVFGVRNSKRGAAGSLMNVLNHPGMNHRVEITEGILAGECAALLCDFYRMPRQVFNAQKKAQSNINPGGSSGGSSGSETPGTSGSATPGSSGGSSGGSAKNTITKALKLRIVRPYNSAEVEKIVADEKNNRERIALEKNKDKVKEACSKHLKVAAYCTTQVERNACLFCKARKLDDKFYQKLRGQFPDAVFWQEIGEIFRQLQKQAAEIYNQSLIELYYEIFIKGKGVANANNVEHYLSDVCYTRAAELFKNAAIASGLRNKIKSNFRLKELRNMKSGLPTTKSDNFPIPLVKQKGGQYTGFEISSHNDDFIIKIPFGRWQVKKVIDKYRPWEKFDFEQVRKSPKPISLLLSTQRRKRNKGWSKDEGTEAEIRKVMNGDYQTSYIEVKRGSKTGEKSAWMLNLSIDVPKIDKGVDPCIIGGIDVGVKSPLVCAINGAFSRYSISDNDLFHFNKRMFARRRILLKKNGHKRAGHGAKNKLKPITIMTEKSKRFRKKLIERWACEIADFFVKNKVGTVQMENLESMKRKEDSYFNIRLRGFWPYAEMQNKIEFKLKQYGIVIRKVAPNNTSKTCSKCGHLNNYFDFEYRKKNKFPHFKCEKCNFKENADYNAALNISNPKLKSTKEEP

SEQ ID NO: 481 - protein, 726 aa, synthetic construct
SEVEFSHEYWMRHALTLAKRARDEREVPVGAVLVLNNRVIGEGWNRTTGLHDPTAHAEIMALRQGGLVMQNYRLIDATLYVTFEPCVMCAGAMIHSRIGRVVFGVRNSKHGAAGSLVNVLNYPGMNHRVEITEGILADECAALLCDFYRMPRQVFNARKKAQSSINSGGSSGGSSGSETPGTSESATPKSSGGSSGGSAKNTITKALKLRIVRPYNSAEVEKIVADEKNNRERIALEKNKDKVKEACSKHLKVAAYCTTQVERNACLFCKARKLDDKFYQKLRGQFPDAVFWQEIGEIFRQLQKQAAEIYNQSLVELYYEIFIKGKGIANASSVEHYLSDVCYTRAAELFKNAAIASGLRNKIKSNFRLKELRNMKSGLPTTKSDNFPIPLVRQKGGQYTGFEISSHNDDFIIKIPFGRWQVKKEIDKYRPWEKFDFEQVRKSPKPISLLLSTQRRKRNKGWSKDEGTEAEIRKVMSGDYQTSYIEVKRGSKTGEKSAWMLNLSIDVPKIDKGVDPSIIGGIDVGVKSPLVCAINNALSRYSISDNDLFHFNKKMFARRRILLKKNRHKRAGHGAKNKLKPITIMTEKSKRFRKKLIERWACEIADFFIKNKVGTVQMENLESMKRKEDSYFNIRLRGFWPYAEMQNKIEFKLKQYGIEIRKVAPNNTSKTCSKCGHLNNYFNFEFRKKNKFPHFKCEKCSFKEDADYNAALNISNPKLKSTKEEP

SEQ ID NO: 482 - protein, 726 aa, synthetic construct
SEVEFSHEYWMRHALILAKRARDEREVPVGAVLVLNNRVIGVGWNRAVGLHDPTAHAEIMALRQGGLVMQNYRLIEATLYVTFEPCIMCAGAMIHSRIGRVVFGVRNSKRGAAGSLMNVLNYPGMNHRVEITEGILVDECAALLCDFYRMPRQVLNAQKKAQSSISPGGSSGGSSGSETPGTSESATPESSGGSSGGSAKNTITKTLKLRIVRPYNSAEVEKIVADEKNNREKIALEKNKDKVREACSKHLKVASYCTTQVERNACLFCKARKLDDKFYQKLRGQFPDAVFWQELGEIFRQLQKQAAEIYNQSLIELYYEIFIKGKGFANASSVEHYLSDVCYTRAAELFKNAAIASGLRGKVKSNFRLKELKNMKSGLPTTKSDNFPIPLVKQKGGQYTGFEIGSHNDDFIIKIPFGRWQAKKEIDKYRPWEKFDFEQVRKSPKPISLLLSIQRRKRNKGWSKDEGTEAEIRKVMNGDYQTSYIEVKRGRKIGEKSAWMLNLSIDVPKIDKGVDPSIVGGIDVGVKSPLVCAINNAFSRYSISDNDLFHFNKKMFARRRVLLRKNRHKRAGHGTKNKLKPITILTEKSGRFRKKLIERWACEIANFFIKNKVGTVQMENLESMKRKEDSYFNIRLRGFWPYAEMQNKIEFKLKQYGIKIRKVAPNNTSKTCSKCGHLNNYFSFEYRKKNKFLHFKCEKCNFKEDADYNAALNISNPKLKSTKEEP

SEQ ID NO: 483 - protein, 726 aa, synthetic construct
SEDEFSHEYWMRHALTLAKRARDEREVPVGAILVLNNRVIGEGWNRAIGLHDPTAHAEIMALRQGGLVMQNYRLTDATLYVTFEPCVMCAGAMIHSRIGRVVFGVRNSKRGAAGSLMNVLNYPGMNHRVEITEGILVDECAALLCDFYRMPRQVLSAQKKAQSSVSSGGSSGGSSGSETPGAGGSVTPKSSGGSSGGSTKNTITKTLKLRIVRPYNSAEVEKIVTDEKNNREKIALEKNKDKVKEACSEHLKVAAYCTTQVERNACLFCKARRLDDKFYQKLRGQFPDAVFWQEISEIFRQLQKQAAEIYNQSLIELYYEIFIKGKGFANASSVEHYLSDVCYTRAAELFKNAAIASGLRGKVKSNFRLKELKNMKSGLPTTKSDNFPIPLVKQKGGQYTGFEISSHNDDFIIKIPFGRWQVKKEIDKYRPWEKFDFEQVRKSPKPISLLLSTQRRKRNKGWSKDEGTEAEIRKVMNGDYQTSYIEVKRGSKIGEKSAWMLSLSIDVPKIDKGVDPSIIGGIDVGVKSPLVCAINNAFCRYSISDNDLFHFNKKMFARRRILLKKSRHKRAGHGAKNKLKPISILTEKSKRFRKKLIERWACEIADFFIKNKVGTVQMENLESMKRKEDSYFNIRLRGFWPYAEMQNKIEFKLKQYGIEIRRVAPNNTSKTCSKCGHLNNYFNFEYRKKNKFPHFKCEKCNFKENADYNAALNISNPKLKSTKEEP

SEQ ID NO: 484 - protein, 726 aa, synthetic construct
SEVEFSHEYWMRHALTLAKRARDEREVPVGAILVLNNRVIGEGWNRAIGLHDPTAHAEIMALRQGGLVMQNYRLIDATLYVTFEPCVMCAGAMVHSRVGRVVFGVRNSKRGAAGSLMNVLDYPGMGHRVEITEGILADECAALLCDFYRMPRRVFNAQKKAQSSINSGGSSGGGSGSETPSTSESTTPKSSGGSSAGSTKNTITKTLKLRIVRPYNSAEVEKIVADEKNSREKVALERNKDKVKEACSEHLKVAAYCTTQVERNACLFCKARKLDDRFYQKLRGQFPDAVFWQETGEIFRQLQRQAAEIYNQSLIELYYEILIKGKGFANASSVEHYLSDVCYTRAAELFKNAAIASGLRGKVKSNFRLKELKSMKSGLPTTKSDNFPIPLVKQKGGQYTGFEISSHNDDFIIKIPFGRWQVKEEIDKYRPWEKFDFEQVRKNPKPISLLLSTQRRKGNKGWSKDEGTEAEIRKVMNGDYQTSYIEVKRGSKIGEKSAWMLNLSIDVPKIDKGVDPSIIGGIDVGVKSPLVCAINNAFSRYSISDNDLFRFNKKVFARRRILLKKNRHKRAGHGTKNKLKPITILTEKSKRFRKKLIERWACEIADFFIKNKVGTVQMENLESMKRKEDSYFNIRLRGFWPYAEMQNKIEFKLKQYGIKIRKVAPNNTSRTCSKCGHLNNYFSFEYRKKNKFPHFKCEKCNFKEDADYNAALNICNPKLKSTKEEP

SEQ ID NO: 485 - protein, 726 aa, synthetic construct
SEVEFSHEYWMRHALTLAKRARDEREVPVGAVLVLNNRVIGEGWNRTIGLHDPTAHAEIMALRQGGLVMQNYRLTDATLYVTFEPCVMCAGAMIHSRIGRVVFGVRNSKRGAAGSLMNVLNYPGMNHCVEITEGILVDECAALLCDFYRMPRQVLNAQKKAQSSISSGGSSGGSSGSETPGASESVTPKSSVGSSAGSTKNTITKTLKLRIVRPYNSAEVEKIVADEKNNRERIALEKNKDKVKEACSKHLKVAAYCTTQVERNACLFCKARKLDDKFYQKLRGQFPDAVFWQETGEIFRQLQRQAAEIYNQSLIELYYEIFIKGKGFANASSVEHYLSDVCYTRAAELFKNAAIASGLRGKVKGNFRLKELKNMKSGLPTTKSDNFPIPLVKQKGGQYTGFEISSHNDDFIIKIPFGRWQAKKEIDKYRPWEKFDFEQVRKSPKPISLLLSTQRRKRNKGWSKDEGTEAEIRKVMNGDYQTSYIEVKRGSKIGEKSAWMLNLSIDVPKIDKGVDPSIIGGIDVGVKSPLVCAINNALSRYSISDNDLFHFNKKMFARRRILLRKNRHKRAGHGARNKLKPITIMTEKSRRFRKKLIERWACEIADFFIKNKVGTVQMENLESMKRKEDSYFNIRLRGFWPYAEMQNKIEFKLKQYGIVVRKVAPNNTSRTCSKCGHLNNYFDFEYRRKYKFPHFKCEKCNFKEDADYNAALNISNPKLKGTKEEP

SEQ ID NO: 486 - protein, 726 aa, synthetic construct
SEVEFSHEYWMRHALTLAKRARDEREVPVGAILVLNNRVIGEGWNRAIGLHDPTAHAEIMALRQGGLVMQNYRLIDATLYVTFEPCVMCAGAMIHSRIGRVVFGVRNSKRGAAGSLMNVLNYPGMNHCVEITEGILVDECAALLCDFYRMPRQVLNAQKKAQSSISFGGSSGGSSGSETPGASGSVTPKSSGGSSAGSTKDTITKTLKLRIVRPYNSAEVEKVVADEKNNREKIAMEKNKDKVKEACSKHLKVASYCTTQVERNACLFCKARKLDDKFYQKLRGQFPDAVFWQELGGILRQLQKQAAEIYNQSLIELYYEIFIKGKGFANASSVEHYLSDVCYTRAAELFKNAAIASGLRGKVKSNFRLKELKNMKSGLPTTKSDNFPIPLVKQKGGQYTGFEISSHNDDFIIKIPFGRWQMKKEIDKYRPWEKFDFEQVRKSPKPISLLLSTQRRKKNKGWSKDEGTEAEIRKVMNGGYQTSYIEVKRGSKIGEKSAWMLNLSIDVPKIDKGVDPSIIGGIDVGVKSPLVCAINNAFSRYSISDNDLFRFNKKMFARRRILLKKNRHKRAGHGAKNKLKPISILTEKSKRFRKKLIERWACEIADFFIKNKVGTVQMENLESMKRREDSYFNIRLRGFWPYAEMQNKIEFKLKQYGIEIRKVAPNNTSKTCSKCGHLNSYFNFEYRKKNKFPHFKCEKCNFKENADYNAALNISNPKLKGTKEEP

SEQ ID NO: 487 - protein, 726 aa, synthetic construct
SEVEFSHEYWMRHALTLAKRARDGREVPVGAVLVLNNRVIGEGWNRAIGLHDPTAHAEIMALRQGGLVMQNYRLIDATLYVTFEPCVMCAGAMVHSRIGRVVFGVRNSKRGAAGSLMNVLDYPGMGHRVEITEGILADECAALLCDFYCMPRQVFNAQKRAQSSINSGGSSGGSSGSETPGTNESATPESSGGGSSGSAKNTITKTLQLRIVRPYNSAEVEKIVADEKNNREKIALEKNKDKVKEACSEHLKVAAYCTTQVERNACLFCKARKLDDKFYQKLRGQFPDAVFWQEIGEIFRQLQRQAAEIYNQSLIELYYEIFIKGKGITNASRVEHYLSDVCYTRAAELFKNAAIASGLRSKVRSNFRLKELKNMKSGLPTTKSDNFPIPLVKQKGGQYTGFEISSHNSDFIIKIPFGRWQVKKEIDKYRPWEKFDFEQVRKSPKPISLLLSTQRRKRNKGWSKDEGTEAEIRKVMNGDYRISYIEVKRGSKVGEKSAWMLSLSIDVPKIDKGVDPSIIGGIDVGVKSPLVCAINNAFSRHSISDNDLFHFNKKMFARRRILLKKNRHKRAGHGAKNKLKPISILTGKSKRFRKKLIERWACEIADFFIKNKVGTVQMENLESMKRKEDSYFNIRLRGFWPYAEMQNKIEFKLKQYGIEIRKVAPNNTSKTCSKCGHLNNYFNFEYRKKNKFPHFKCEKCNFKENADYNAALNISNPKLKSTKGEP

SEQ ID NO: 488 - protein, 726 aa, synthetic construct
SEVEFSHEYWMRHALTLAKRARDEREVPVGAVLVLSNRVIGEGWNRAIGLHDPTAHAEIMALRQGGLVMQNYRLTDATLYVTFEPCVMCAGAMVHSRIGRVVFGVRNSKRGAAGSLMNVLNYPGMGHRVEITEGILADECAALLCDFYRMPHQVFSARKKAQSSINPGGSSGGSGGSETPGTSESATPESSGGSSGSSAKNTITKTLKLRIVRPYNSAEVEKIVADEKNNREKIALEKNKDKVKEACSKHLKVATYCTTQVERNACLFCKARRLDDKFYQKLRGQFPDAVFWQEIGEIFRQLQKQAAEIYNQSLVELYYEILIKGKGIANASSVEHYLSDVCYTRAAELFKNAAIASGLRNKIKSNFRLKELRNMKSGLPTTKSDNFPIPLVRQKGGQYTGFEISNHDGDFIIKIPFGRWQVKKEINKYRPWEKFDFEQVRKSPKPISLLLSTQRRKRNKGWSKDEGTEAEIRKVMNGDYQTSYIEVKRGSKIGEKSAWMLNLSIDVPKIDKGVDPSIIGGIDVGVKSPLVCAIDNAFSRYSISDNDLYHFNKKMFAKRRILLKKNRHKRAGHGAKNKLKPISILTEKSERFRKKLIERWACEIADFFIKNKVGTVQMENLESMKRREDSYFNTRLRGFWPYAEMQNKIEFKLKQYGIEIRKVAPNNTSKTCSKCGHLNNYFSFEYRKKNKFPHFKCEKCNFKENADYNAALNISNPKLKSTKEES

SEQ ID NO: 489 - protein, 726 aa, synthetic construct
SEVEFSHEYWMRHALTLAKRARDEREVPVGAVLVLNNRVIGEGWNRAIGLHDPTAHAEIMALRQGGLVMQNYRLIDATLYVTFEPCVMCAGAMIHSRIGRVVFGVRNNKRGAAGSLMNVLNYPGMNHRVEITEGILADECAALLCDFYCMPRQVLNAQKKARSCINSGGSSGGSSGSETPGTSESVTPESSGGSSGGSAKNTITKTLKLRIVRPYNSAEVEKIVADEKDNRERIALEKNKGKVKEACSKHLKVAAYCTTQVERNACLFCKARKLDDKFYQELRGQFPDAVFWQEIGEIFRQLQKQAAEIYNQSLIELYYEIFIKGKGFANASSVEHYLSDVCYTRAAELFKNAAIASGLRGKVKSNFRLKELKNMKSGLPTTKSDNFPIPLVKQKGGQYTGFEISSHNDDFIIKIPFGRWQVKKEIDKYRPWEKFDFEQVRKSPKPISLLLSTQRRKRNKGWSKDEGTEAEIRKVMNGDYQTSYIEVKRGNKIGEKSAWMLNLSIDVPKIDKGVDPCIIGGIDVGVKSPLVCAINNAFSRYSISDNDLFHFNKKMFARRRILLKKNGHKRAGHGAKNKLKPITIMTEKSKRFRRKLIERWACEIADFFIKNKVGTVQMENLESMKRREDSYFNIRLRGFWPYAEMQSKIEFKLKQYGIKIRKVAPNNTSRTCSKCGHLNNYFNFEFRKKNKFPHFKCEKCNFKEDADYNAALNISDPKLKSTKEEP

SEQ ID NO: 490 - protein, 726 aa, synthetic construct
SEVEFSHEYWMRHALTLAKRARDEREVPVGAVLVLNDRAIGEGWNRAIGLHDPTAHAEIMALRQGGLVMQNYRLTDATLYVTFEPCVMCAGAMIHSRIGRVVFGVRNSKHGAAGSLMNVLNYPGMNHRVEITEGILADECAALLCDFYRMPRQVFSARKKAQSSINSGGSSGGNSGNKTPGTSESATPESSGGSSGSSAKNTITKTLKLRIVRPYNSAEVEKIVADEKNNREKIALEKNKDKVREACSKHLKVASYCTTQVERNACPFCKARKLDDKFYQKLRGQFPDAVFWQELGEILRQLQKQAAEIYNQSLIELYYEIFIKGRGFANASSVEHYLSDVCYTRAAELFKNAAIASGLRGKVKSNFRLKELKNMKSGLPTTKSDNFPIPLVKQKGGQYTGFEISSHNDDFIIKIPFGRWQVKEEIDKYRPWEKFDFEQVRKNPKPISLLLSTQRRKRNKGWSKDEGTEAEIRKVMNGDYQTSYIEVKRGSKIGEKSAWMLNLSIDVPKIDKGVDPSIIGGIDVGVKSPLVCAINNALSRYSISDNDLFHFNKKMFARRRILLRKNRHKRAGHGAKNKLKPITMMTEKSKRFRKKLIERWACEIADFFIKNKVGTVQMENLESMKRKEDSYFNIRLRGFWPYAEMQNKIEFKLKQYGIVVRKVAPNNTSKTCSKCGHLNNYFNFEYRKKNKFPHFKCEKCNFKENADYNAALNISNPKLKSTKEEP

SEQ ID NO: 491 - protein, 726 aa, synthetic construct
SEVEFSHEYWMRHALTLAKRARDEREVPVGAVLVLNNRVIGEGWNRAIGLHDPTAHAEIMALRQGGLVMQNYRLTDATLYVTFEPCVMCAGAMVHSRIGRVVFGVRNSKRGAAGSLMNVLNYPGMNHRVEITEGILADECAALLCDFYRMPRQIFNAQKKAQSSINPGGSSGGSSGSETPGTSESATPESSGGSSGSSAKNTITKTLKLRIVRPYNNAEVEKIVADEKNNREKIALEKNKDKVKEACSKHLKVAAYCTTQVERNACLFCKARRLDDKFYQKLRGQFPDAVFWQEIGEIFRQLQKQAAEVYNQSLVELYYEILIKGKGIANASSVEHYLSDVCYTRAAELFKNAAIASGLRNKIKSNFRLKELRNMKSGLPTTKSDNFPIPLVRQKGGQYTGFEISNHDGDFIIKIPFGRWQVKKEINKHRPWEKFDFEQVRKSPKPISLLLSTQRRKRNKGWSKDEGTEAEIRKVMNGDYQTSYIEVKRGSKIGEKSAWMLNLSIDVPKIDKGVDPSIIGGIDVGVKSPLVCAINNALSRYSISDNDLFHFNKKMFARRRILLRKNRHKRAGHGAKNKLKPITIMTEKSKRFRKKLIERWACEIADFFIKNKVGTVQMENLESMKRKEDSYFNIRLRGFWPYAEMQNKIEFKLKQYGIVVRKVAPNNTSKTCSKCGHLNNYFNFEYRKKNKFPHFKCEKCNFKENADYNAALNISNPKLKSTKGEP

SEQ ID NO: 492 - protein, 726 aa, synthetic construct
SEVEFSHEYWMRHALTLAKRARDEREVPVGAVLVLNNRVIGVGWNRAIGLHDPTAHAEIMALRQGGLVMQNYRLTDATLYVTFEPCVMCAGAMVHSRIGRVVFGVRNSKRGAAGSLMNVLNYPGMSHCVEITEGILVDECAALLCDFYRMPRQVFNARKKAQSSINPSGSSGGSSGSVTPGTSESATPESSGGGSGGSAKNTITKTLQLRIVRPYNSAEVEKIVTDEKNNREKIALEKNKDKVKEACSKHLKMASYCTTQVERNACLFCKARKLDDKFYQKLRGQFPDAVFWQELGGIFRQLQKQAAEIYNQSLIELYYEIFIKGKGITNASRVEHYLSDVCYTRAAELFKNAAIASGLRSKVRSNFRLKELKNMKSGLPTTKSDNFPIPLVKQKGGQYTGFEISSHNDDFIIKIPFGRWQVKEEIDKYRPWEKFDFEQVRKNPKPISLLLSTQRRKRNKGWSKDEGTEAEIRKVMNGDYQTSYIEVKRGSKIGEKSAWMLNLSIDVPKIDKGVDPSIIGGIDVGVKSPLVCAINNAFSRYSISDNDLFRFNKKVFARRRILLKKNRHKRAGHGTKNKLKPITILTEKSGRFRKKLIERWACEIANFFIKNKVGTVQMENLESMKRKGDSYFNIRLRGFWPYAEMQNKIEFKLKQYGIKIRKVAPNNTSKTCSKCGHLNNYFSFEYRKKNKFPHFKCEKCNFKEDADYNAALNISNPKLRSTKEEP

SEQ ID NO: 493 - protein, 726 aa, synthetic construct
SGVEFSHEYWMRHALTLAKRARDEREVPVGAILVLNNRVIGEGWNRAIGLHDPTAHAEIMALRQGGLVMQNYRLIDATLYVTFEPCVMCAGAMIHSRIGRVVFGVRNNKHGAAGSLVNVLNYPGMNHRVEITEGILADECAALLCDFYRMPRQVFNARKKAQSSINPGGSSGGSSGSETPGTSESATPESSGGSPGGSAKNTITKTLKLRIVRPYNCAEVEKIVADEKNNREKIALEKNKDKVKEACSEHLKVAAYCTTQVERSACLFCKARKLDDKFYQKLRGQFPDAVSWQEIGEIFRQLQKQAAEIYNQSLIELYYEIFIKGKGFANASSVEHYLSDVCYTRAAELFKNAAIASGLRGKVKSNFRLKELKNMKSGLPTTKSDNFPIPLVKQKGGQYTGFEISSHNDDFIIKIPFGRWQVKKEIDKYRPWEKFDFEQVRKSPKPISLLLSTQRRKRNKGWSKDEGTEAEIRKVMNGDYQTSYIEVKRGSKAGEKSAWMLNLSIDVPKIDRGVDPSIIGGIDVGVKSPLVCAINNAFSRYSISDNDLFHFNKKMFARRRILLGKNRHKRAGHGVKNKLKPITILTEKSGRFRKKLMERWACEIADFFVKNKVGTVQMENLESMKRKEDSYFNIRLRGFWPYAEMQNKIEFKLKQYGIKVRKVAPNNTSKTCSKCGHLNSYFNFEYRKKNKFPHFKCEKCNFRENADYNAALNISNPKLRSTKEEP

SEQ ID NO: 494 - protein, 726 aa, synthetic construct
SEVEFSHEYWMRHALSLAKRARDEREVPVGAVLVLNNRIIGEGWNRAIGQHDPTAHAEIMALRQGGLVMQNYRLTDATLYVTFEPCVMCAGAMVHSHIGRVVFGVRNSKRGAAGSLMNVLNYPGVNHCVEITEGILVDECAALLCDFYRMPRRVFNAQKKAQSSISSGGSSGGCSGSEMPGASESVTPKSSGGSSAGSTKNTITKTLKLRIVRPYNSAEVEKIVADEKNNREKIALEKNKDKVREACSKHLKMASYCTTQVERNACLFCKARRLDDKFYQKLRGQFPDAVFWQEIGEIFRQLQKQAAEIYNQSLVELYYEILIKGKGIANASSVEHYLSDVCYTRAAELFKNAAIASGLRGKVKSNFRLKELKNMRSGLPTTKSDNFPIPLVKQKGGQYAGFEISSHNSDFIIKIPFGRWQVKEEIDKYRPWEKFAFEQVRKNPKPISLLLSTQRRKGNKGWSKDEGTEAEIRKVMNGDYQTSYIEVKRGSKIGEKSAWMLNLSIDVPKIDKGVDPSIIGGIDVGVKSPLVCAINNAFSRYSISDNDLFHFNKKMFARRRILLKKNRHRRAGHGAKNKLKPITILTEKSKRFRKKLIERWACEIADFFIKNKVGTVQMENLESMKRKEDSYFNIRLRGFWPYAEMQNKIEFKLKQYGIKIRKVAPNNTSRTCSECGHLNNYFSFEYRKKNKFPHFKCEKCNFKEDADYNAALNISNPKLKGTKEEL

SEQ ID NO: 495 - protein, 726 aa, synthetic construct
SEVEFSHEYWMRHALTLAKRARDEHEVPVGAVLVLNNRVIGEGWNRAIGLHDPTAHAEIMALRQGGLVMQNCRLVDATLYVTFEPCVMCAGALIHSRIGRVVFGVRNSKRGAAGSLMNVLNHPGMNHRVEITEGILAGECAALLCDFYRMPRQVFNARKKAQSTINSGGSSGGSSSSETPGISGSATPEGSGGSSGGSTKNTITKTLKLRIVRPYNSAEVEKIVADEKNNREKIALEKNKDKVKEACSKHLKVASYCTTQVERNACLFCKARKLDDKFYQKLRGQFPDAVFWQELGEIFRQLQKQAAEIYNQSLIELYYEIFIKGRGFANAGSVEHYLSDVCYTRAAELFKNAAIASGLRGKVKSNFRLKELKNMKSGLPTTKSDNFPIPLVKQKGGQYTGFEISSHNDDLIIKIPFGRWQVKKEIDKYRPWEKFDFEQVRKSPKPISLLLSTQRRKRNKGWSKDEGTEAEIRKVMNGDYQTSYIEVKRGSKIGEKSAWMLNLSIDVPKIDKGVDPSIIGGIDVGVQSPLVCAINNAFSRYSISDNDLFHFNKKMFARRRILLKKNRHKRAGHGAKNKLRPITIMTEKSKRFRKKLIERWACEIADFFIKNKVGTVQMENLESMKRKEDSYFNIRLRGFWPYAEMQNKIEFKLKQYGIVVRKVAPNNTSKTCSKCGHLNNYFSFEYRKKNKFPHFKCEKCNFKENADYNAALNISNPKLKSTKEEP

SEQ ID NO: 496 - protein, 726 aa, synthetic construct
SEVEFSHEYWMRHALTLAKRARDEREVPVGAVLVLNNRVIGEGWNRAIGLHDPTAHAEIMALRQGGLVMQNYRLTDATLYVTFEPCVMCAGAMIHSRIGRVVFGVRNSKRGAAGSLMNVLNYPGMNHCVEITEGILVDECAALLCDFYRMPRQVLNAQKKAQSSISSGGSSGGSSCSETPGASESVTPKSSGGRSAGTTKNTITKTLKLRIVRPYNSAEVEKIVADEKNSREKIALEKNKDKVKEACSEHLKVAAYCTTQVERNACLFCKARKLDDRFYQKLRGQFPDAVFWQEIGEIFRQLQKQAAEIYNQSLIELYYEIFIKGKGFANASSVEHYLSDVCYTRAAKLFKNAAIASGLRGKVKSNFRLKELKNMKSGLPTTKSDNFPIPLVKQKGGQYTGFEVSSHNDDFIIKIPFGRWQVKKEIDKYRPWEKFDFEQVRKSPRPISLLLSTQRRKRNKGWSKDEGTEAEIRKVMNGDYQTSYIEVKRGSKIGEKSAWMLNLSIDVPKIDKGVDPSIIGGIDVGVKSPLVCAIDNAFSRYSISDNDLYHFNKKMFAKRRILLKKNRHKRAGHGAKNKLKPISILTEKSERFRKKLIERWACEIADFFIKNKVGTVQMENLESMKRREDSYFNTRLRGFWPYAEMQNKIEFKLKQYGIEIRKVAPNNTSKTCSKCGHLNNYFNFEYRKKNKFPHFKCEKCNFKENADYNAALNISNPRLKSTKEEP

SEQ ID NO: 497 - protein, 726 aa, synthetic construct
SEVEFSHEYWMRHALTLAKRARDEREVPVGAILVLNNRVIGEGWNRAIGLHDPTAHAEIMALRQGGLVMQNYRLTDATLYVTFEPCVMCAGAMIHSRIGRVVFGVRNSKRGAAGSLMNVLNYPGMNHCVEITEGILVDECAALLCDFYRMPRQVLNAQKKAQSSISSGGSSGGSGGGETPGASESVTPKNSGGSSAGSTKNTITKTLKLRIVRPYNSAEVEKIVADEKNSREKIALEKNKDKVKEACREHLKVAAYCTTQVERSACLFCKARKLDDKFYQKLRGQFPDAVFWQEIGEIFRQLQKQAAEVYNQSLVELYYEILIKGKGIANASSVEHYLSDVCYTRAAELFKNAAIASGLRNKIKSNFRLKELRNMKSGLPTTKSDNFPIPLVRQKGGQYTGFEISNHDGDFIIKIPFGRWQVKKEINKHRPWEKFDFEQVRKSPKPISLLLSTQRRKRNKGWSKDEGTEAEIRKVMNGDYQTSYIEVKRGSKIGEKSAWMLNLSIDVPKIDKGVDPSIIGGIDVGVKSPLVCAINNAFSRYSISDNDLFRFNKKMFARRRILLKRNRHKRAGHGAKNKLKPITILTGKSERFRKKLIERWACEIADFFIKNRVGTVQMENLESMKRKEDSYFNIRLRGFWPYAEMQNKIEFKLKQYGVKIRKVAPNNTSRTCSKCGHLNNYFSFEYRKKNKFPHFKCEKCNFKENADYNAALNISNPKLMSTKEEP

SEQ ID NO: 498 - protein, 726 aa, synthetic construct
SEVEFSHEYWMRHALTLAKRARDEREVPVGAVLVLNNRVIGEGWNRTTGLHDPTAHAEIMALRQGGLVMQNCRLVDATLYVTFEPCVMCAGAMIHSRIGRVVFGVRNSKRGAAGSLMNVLNYPGMNHRVEITEGILAGECAALLCDFYRMPRQVFNAQKKAQSTINSGGSSGGSSGSETPGTSGSATPESSGGSSGGSAKNTITKTLKLRIVRPYNSAEVEKIVADEKNNREKIALEKNKDKVKEACSEHLKVAAYCTTQVERNACPFCKARKLDDKFYQKLRGQFPGAVFWQEIGEIFRQLQKQAAEIYNQSLIELYYEIFIKGKGIANASSVEHYLSDVCYTRAAELFKNAAIASGLRNKVKSNFRLKELRSMKSGLPTTKSDNFPIPLVRQKGGQYTGFEISNHNSDFIIKIPFGRWQAKEEIDKYRPWEKFDFEQVRKSPKPISLLLSTQRRKRNRGWSKDESTEAEIKKVMNGDYQTSYIEVKRGSKVGEKSAWMLNLSIDVPKIDKGVDPSIIGGIDVGVKSPLVCAINNAFSRYSISDNDLYRFNKKMFARRRILLKKSKHKRAGHGAKNKLKPITILTEKSGRFRKKLIERWACEIADFFIKNKVGTVQMENLEGMKRKEDSYFNIRLRGFWPYAEMQNKIEFKLKQYGIEIRKVAPNNTSKTCSKCGHLNNYFNFEYRKKNKFPHFKCEKCNFKENADYNAALNISNPKLKSTKEGP

SEQ ID NO: 499 - protein, 726 aa, synthetic construct
SEVEFSHEYWMRRALTLAKRARDEREVPVGAVLVLNNRVIGVGWNRAVGLHDPTAHAEIMALRQGGLVMQNYRLIEATLYVTFEPCIMCAGAMIHSRIGRVVFGARNSKRGAAGSLMNVLNYPGMNHRVEITEGILADECAALLCDYYRMPRQVFNARKKAQSSINSGGSSDGGSGSETPGTSESATPESSGGSSGGSAKNTITKTLKLRIVRPFNSAEVEKIVADEKNNREKIALEKNKDKVREACSEHLKVAAYCTTQVERSACLFCKARKLDDKFYQKLRGQFPDAVFWQEIGEIFRQLQKQAAEIYNQSLIELYYEIFIKGRGFANASSVEHYLSDVCYTRAADLFKNAAIASGLRGKVKGNFRLKELKNMKSGLPTTKSDNFPIPLVKQKGGQYTGFEISSHNDDFIIKIPFGRWQVKKEIDKYRPWEKFDFEQVRKSPKPISLLLSTQRRKRNKGWSKDEGTEAEIRKVMNGDYQTSYIEVKRGSRIGEKSAWMLCLSIDVPKIDRGVDPSIIGGIDVGVKSPLVCAINNALSRYSISDNDLFHFNKKMFARRRILLKKNRHRRAGHGARNKLKPITALTEKSKRFRKKLIERWACEIADFFIKNKVGTVQIENLESMKRREDSYFNIRLRGFWPYAEMQNKIEFKLKQYGIEIRKVAPNNTSKTCSKCGHLNNYFNFEYRKRNKFPHFKCEKCNFKENADYNAALNISNPKLKSPKEES

SEQ ID NO: 500 - protein, 726 aa, synthetic construct
SEVEFSHEYWMRHALTLARRARDEREVPVGAILVLNNRVIGEGWNRAIGLHDPTAHAEIMALRQGGLVMQNYRLIDATLYVTFEPCVMCAGAMIHSRIGRVVFGVRNSKHGAAGSLMNVLNYPGMNHRVEITEGILADECAALLCDFYRMPRQVFNARKKAQSSINSGGSSGGSSGSETPGASGSVTPKSSGGSSAGSTKDTITKTLKLRIVRPYNSAEVEKIVADEKNSREKIALEKNKDKVREACSKHLKVASYCTTQVERNACPFCKARKLDDKFYQKLRGQFPDAVFWQELGEILRQLQKQAAEIYNQSLIELYYEIFIKGRGFANASSVEHYLSDVCYTRAAELFKNAAIASGLRGKVKSNFRLKELKNMRSGLPTTKSDNFPIPLVKQKGGQYAGFEISSHNDDFIIKIPFGRWQVKKEIDKYRPWEKFDFEQVRKSPKPISLLLSTRRRKRNKGWSKDEGTEAEIRKVMNGDYQTSYIEVKRGSKTGERSAWMLNLSIDVPKIDKGVNPSIIGGIDVGVKSPLVCAINNAFSRYSISDNDLFRFNKKMFARRRILLGKNRHKRAGHGVKNKLKPITILTEKSGRFRKKLIERWACEIADFFIKNKVGTVQMENLESMKRKEDSYFNIRLRGFWPYAEMQNKIEFKLKQYGIVVRKVAPNNTSKTCSQCGHLNNYFNFEYRKKNKFPYFKCEKCNFKENADYNAALNISNPQLKSTKGEP

SEQ ID NO: 501 - protein, 726 aa, synthetic construct
SEVEFSHEYWMRHALTLARRARDGREVPVGAVLVLNNRVIGEGWNRAIGLHDPTAHAEIMALRQGGLVMQNYRLIDATLYVTFEPCVMCAGAMVHSRIGRVVFGVRNSKRGAAGSLMNVLDYPGMGHRVEITEGILADECAALLCDFYRMPRQVFNARKKAQSSINSGGSSGGSSGSETPGTSGSATPVSSSGSSGGSAKNTITKTLKLRIVRPYNSAEVEKIVADEKNNREKIALEKNKDKVKEACSEHLKVATYCSTQVERNACLFCRARRLDDKFYQKLRGQFPDAVFWQEIGEIFRQLQKQAAEIYNQSLVELYYEILIKGKGIANASSVEHYLSDVCYTRAAELFKNAAIASGLRNKIKSNFRLKELRNMKSGLPTTKSDNFPIPLVRQKGGQYTGFEISNHDGDFIIKIPFGRWQVKKEINKHRPWEKFDFEQVRRSPKPISLLLSTQRRKRNKGWSKDEGTEAEIRKVMNGDYQTSYIEVKRGSKIGEKSAWMLSLSIDVPKIDKGVDPSIIGGIDVGVKSPLVCAINNAFCRYSISDNDLFHFNKKMFARRRILLKKSRHKRAGHGAKNKLKPISILTEKSKRFRKKLIERWACEIADFFIKNKVGTVQMENLESMKRKEDSYFNIRLRGFWPYAEMQNKIEFKLKQYGIEIRKVAPNNTSKTCSKCGHLNNYFNFEYRKKNKFPHFKCEKCNFKENADYNAALNISNPKLKSTKEEP

SEQ ID NO: 502 - protein, 726 aa, synthetic construct
SEVEFSHEYWMRHALTLAKRARDEREVPVGAVLVLNNRVIGEGWNRAIGLHDPTAHAEIMALRQGGLVMQNHRLVDATLYVTFEPCVMCAGAMIHSRIGRVVFGVRNSKRGAAGSLMNVLNYPGMNHCVEITEGILVDECAALLCDFYRMPRQVLSAQKKAQSSISSGGSSGGSSGSETPGASGSVTPKSSVGSSAGSTKNTITKTLKLRIVRPYNSAEVEKIVADEKNNREKIALEKNKDKVKEACSKHLKVAAYCTTQVERNACLFCKARKLDDKFYQKLRGQFPDAVFWQEIGEIFRQLQKQAAEIYNQSLIELYYEIFIKGKGFANASSVEHYLSDVCYTRAAELFKNAAIASGLRGKVKSNFRLKELKNMKSGLPTTKSDNFPIPLVKQKGGQYTGFEISSHNDDFIIKIPFGRWQVKKEIDRYRPWEKFDFEQVRKSPKPISLLLSTQRRKRSKGWSKDEGTEAEIRKVMSGDYQTSYIEVKRGSKTGEKSAWMLNLSIDVPKIDKGVDPSIIGGIDVGVKSPLVCAINNALSRYSISDNDLFHFNKKMFARRRILLKKNRHKRAGHGAKNKLKPISILTEKSERFRKKLIERWACEIADFFIKNKVGTVQMENLESMKRREDSYFNIRLRGFWPYAKMLNKIEFKLKQYGIKIRKVAPNNTSKTCSKCGHLNNYFNFEYRKKNKFPHFKCEKCNFKENADYNAALNISNPKLKSTKGES

SEQ ID NO: 503 - protein, 726 aa, synthetic construct
SEVEFSHEYWMRHALTLAKRARDEREVPVGAILVLNNRVIGEGWNRAIGLNDPTAHAEIMALRQGGLVMQNYRLIDATLYVTFEPCVMCAGAMIHSRISRVVFGVRNNKHGAAGSLVNVLNYPGMNHRVEITEGILADECAALLCDFYRMPRQVFNARKKAQSSINPGGSSGSSSGSETPGTSESATPESSGGSSGGSAKNTITKTLKLRIVRPYNSAEVEKIVADEKNNREKIALEKNKGKVKEACSKHLKVAAYCTTLVERNACLFCKARRLDDKFYQKLRGQFPDAVFWQEIGEIFRQLQKQAAEIYNQSLIELYYEIFIKGKGFANASSVEHYLSDVCYTRAAELFKNAAIASGLRGKVKSNFRLKELKNMKSGLPTTKSDNFPIPLVKQKGGQYTGFEISSHNDDFIIKIPFGRWQVKKEIDKYRPWEKFDFEQVRKSPKPISLLLSTQRRKRNKGWSKDEGTEAEIRKVMNGDYQTSYIEVKRGSKIGEKSAWMLSLSIDVPKIDKGVDPSIIGGIDVGVKSPLVCAINNALSRYSISDNDLFRFNKKMFARRRILLKKNRHKRAGHGAKNKLKPISVLTEKSGRFRKKLIERWACEIADFFIKNKVGTVQMENLESMKRKEDSYFNIRLRGFWPYAEMQNKIEFKLKQYGIEIRKVAPNNTSKTCSKCGHLNNYFNFEYRRKNKFPHFKCEKCNFKENADYNAALNISNPKLKSTKEEP

SEQ ID NO: 504 - protein, 726 aa, synthetic construct
SEVEFSHEYWMRHALTLAKRARDEREVPVGAVLVLNDRVIGEGWNRAIGLHDPTAHAEIMALRQGGLVMQNYRLIDATLYVTFEPCVMCAGAMIHSRIGRVVFGVRNSKHGAAGSLVNVLNYPGMNHRVEITEGILADECAALLCDFYRMPRQVFNARKKAQSSINPSGSSGGSSGSVTPGTSESATPESSGGGFGGSAKNTITKTLQLRIVRPYNSAEVEKIVADEKNNREKIALEKNKDKVKEACSKHLKVASYCTTQVERNACPFCKARKLDDKFYQKLRGQFPDAVFWQELGEIFRQLQKQAAEIYNQSLIELYYEIFIKGRGFANASSVEHYLSDVCYTRAAELFKNAAIASGLRGKVKGNFRLKELKNMKSGLPTTKSDNFPIPLVKQKGGQYTGFEISSHNDDFIIKIPFGRWQVKKEIDKYRPWEKFDFEQVRKGPKPISLLLSTQRRKRNKGWSKDEGTEAEIRKVMNGDYQTSYIEVKRGSKTGEKSAWMLNLSIDVPKIDKGVDPSIIGGIDVGVKSPLVCAINNAFSRYSISDNDLFRFNKKMFARRRILLKKNRRKRAGHGAKNKLKPISILTEKSKRFRKKLIERWACEIADFFIKNKVGTVQMENLESMKRREDSYFNTRLRGFWPYAEMQNKIEFKLKQYGIEIRKVAPNNTSKTCSKCGHLNNYFNFEYRKMNKFPYFKCEKCNFKENADYNAALNISNPKLRSTKEEP

SEQ ID NO: 505 - protein, 726 aa, synthetic construct
SEVEFSHEYWMRYALTLAKRARDEREVPVGAVLVLNNRVIGEGWNRAIGLHDPTAHAEIMALRQGGLVMQNYRLVDATLYVTFEPCVLCAGAMVHSRIGRVVFGVRNSKRGAAGSLMNVLNYPGMNHRVEITEGILADECAALLCDYYRMPRQVFNARKKAQSSINSGGSSGGSSGSETPGTGESATPESSGGSSGGSAKNTITKTLRLRIVRPYNSAEVEKIVADEKDNREKIALEKNKDKVKEACSEHLKVAAYCTTQVERNACLFCRARKLDDKFYQKLRGQFPDAVFWQEIGEIFRQLQKQAAEIYNQSLIELYYEIFIKGKGFANASSVEHYLSDVCYTRAAELFKNAAIASGLRGKVKSNLRLKELKNMKSGLPTTRSDNFPIPLVKQKGGQYTGFEISSHNDDFIIKIPFGRWQVKKEIDKYRPWEKFDFEQVRKSPKPISLLLSTQRRKRNKGWGKDEGTEAEIRKVMNGDYRTSYIEVKRGSKIGEKSAWMLSLSIDVPKIDKGVDPSIIGGIDVGVKSPLVCAINNAFSRYSISDNDLFHFNKKMFARRRILLKKNRHKRAGHGAKNKLKPISILTGKSERFRKKLIERWACEIADFFIKNRVGTVQMENLESMKRKEDSYFNIRLRGFWPYAEMQNKIEFKLKQYGIVVRKVAPNNTSKTCSKCGHLNNYFNFEYRKKNKFPHFKCEKCNFKENADYNAALNISNPKLKSTKEEP

SEQ ID NO: 506 - protein, 726 aa, synthetic construct
SEDEFSHEYWMRHALTLAKRARDEREVPVGAVLVLNNRVIGEGWNRAIGLHDPTAHAEIMALRQGGLVMQNYRLTDATLYVTFEPCVMCAGAMIHSRIGRVVFGVRNSKRGAAGSLMNVLNYPGMNHCVEITEGILVDECAALLCDFYRMPRQVLNAQKKAQSSISPGGSSGGSSGSETPGASGSVTPKSSGGSSAGSTKDTITKTLKLRIVRPYNSAEVEKIVADEKDNREKIALEKNKDKVKEACSKHLKVASYCTTQVERNACPFCKARKLDDKFYQKLRGQFPDAVFWQELGEILRQLQKQAAEIYNQSLIELYYEIFIKGRGFANASSVEHYLSDVCYTRAAELFKNAAIASGLRGKVKSNFRLKELKNMKSGLPTTKSDNFPIPLVKQKGGQYTGFEISSHNDDFVIKIPFGRWQVKEEINKYRPWEKFDFEQVRKSPKPISLLLSTQRRKRNKGWSKDEGTEAEIRKVMNGDYQTSYIEVRRGSKIGERSAWMLNLSIDVPKIDKGVNPSIIGGIDVGVKSPLVCAINNAFSRYSISDNDLFRFNKKMFARRRILLGKNRHKRAGHGVKNKLKPITILTEKSGRFRKKLIERWACEIADFFVKNKVGTVQMENLESMKRKEDSYFNIRLRGFWPYAEMQNKIEFKLKQYGIEIRKVAPNNTSKTCSKCGHLNSYFNFEYRKKNKFPHFKCEKCNFREDADYNAALNISNPKLRSTKEEP

SEQ ID NO: 507 - protein, 726 aa, synthetic construct
SEVEFSHEYWMRHALTLAKRARDEREVPVGAILVLNNRVIGVGWNRAVGLHDPTAHAEIMALRQGGLVMQNYRLIEATLYVTFEPCIMCAGAMIHSRIGRVVFGVRNSKRGAAGSLMNVLNYPGMNHRVEITEGILADECAALLCDYYRMPRQVLNARKKAQSSTNSGGSSDGGSGSETPGTSESATPESSGGSSGGSAKNTITKTLTLRIVRPYNSAEVEKIVADEKNNREKIALEKNKDKVKEACSEHLKVAAYCTTQVGRNACLFCKARKLDDKFYQKLRGQFPDAVFWQELGEIFRQLQRQAAEIYNQSLIELYYEIFIKGKGFANASSVEHYLSDVCYTRAAELFKNAAIASGLRGKVKGNFRLKELKNMKSGLPTTKSDNFPIPLVKQKGGQYTGFEISSHNDDFIIKIPFGRWQAKKEIDKYRPWEKFDFEQVRKSPKPISLLLSTQRRKRNKGWSKDEGTEAEIRKVMNGDYQTSYIEVKRGSKTGEKSAWMLNLSIDVPKIDKGVDPSIIGGIDVGVKSPLVCAINNALSRYSISDNDLFRFNKKMFARRRILLKKNRHKRAGHGARNKLKPITVLTEKSERFRKKLIERWACEIANFFIKNKVGTVQMENLESMKRREDSYFNIRLRGFWPYAEMQSKIEFKLKQYGIKIRKVAPNNTSKTCSKCGHLNNYFNFEYRKKNKFPHFKCEKCNFKENADYNAALNISNPKLKSTKEEP

SEQ ID NO: 508 - protein, 726 aa, synthetic construct
SEVEFSHEYWMRHALTLAKRARDEREVPVGAVLVLNNRVIGEGWNRAIGLHDPTAHAEIMALRQGGLVMQNYRLTDATLYVTFEPCVMCAGAMIHSRIGRVVFGVRNSKRGAAGSLMNVLNYPGMNHCVEITEGILVDECAALLCDFYRMPRQVLNAQKKAQSSISSGGSSGGSSCSETPGASESATPKSSGGSSAGSTKNTITKTLKLRIVRPYNSAEVEKIVADEKNSREKTALEKNKDKVKEACSKHLKVAAYCTTQVERSACLFCRARKLDDKFYQKLRGQFPEAVFWQEIGEIFRQLQKQAAEIYNQSLIELYYEIFIKGKGFANASSVEHYLSDVCYTRAAELFKNAAIASGLRGKVKSNFRLKELKNMKSGLPTTKSNNFPIPLVKQKGGQYTGFEISSHNDDFIIKIPFGRWQVKKEIDKYRPWEKFDFEQVRKSPKPISLLLSTQRRKRNKGWSKDEGTEAEIRKVMNGDYQTSYIEVKRGSKTGEKSAWMLSLSIDVPKIDKGVDPSIIGGIDVGVKSPLVCAINNAFSRYSISDNDLFRFNKKMFARRRILLKKNRHKRAGHGAKNKLKPISILTRKSERFRRKLIERWACEIADFFIKNKVGTVQMENLESMKRKEDSYFNIRLRGFWPYAEMQNKIEFKLKQYGIEIRKVAPNNTSKTCSKCGHLNNYFNFEYRKKNKFPHFKCEKCNFKENADYNAALNISNPKLKSTKEEP

SEQ ID NO: 509 - protein, 726 aa, synthetic construct
SEVEFSHEYWMRHALTLAKRARDEREVPVGAVLVLNNRAIGEGWNRAIGLHDPTAHAEIMALRQGGLVMQNYRLTDATLYVTFEPCVMCAGAMIHSRIGRVVFGVRNSKRGAAGSLMNVLNYPGMNHCVEITEGILVDECAALLCDFYRMPRQVLNAQKKAQSSISSGGSSGGCSGSEMPGASESVTPKSSGGSSAGSTKNTITKTLKLRIVRPYNSAEVEKIVADEKNSREKIALERNKDKVKEACSEHLKVAAYCTTQVERNACLFCKARRLDDKFYQKLRGQFPDAVFWQEIGEIFRQLQKQAAEIYNQSLVELYYEILIKGKGIANASSVEHYLSDVCYTRAAELFKNAAIASGLRNKIKSNFRLKELRNMRSGLPTTKSDNFPIPLVRQKGGQYTGFEISNHDGDFIIKIPFGRWQVKKEINKHRPWEKFDFEQVRKSPKPISLLLSTQRRKRNKGWSKDEGTEAEIRKVMNGDYQTSYIEVKRGSKIGEKSAWMLNLSIDVPKIDKGVDPSIIGGIDVGVKSPLVCAINNSSSRYSICDNDLFRFNKKMFARRRILLKKNRHKRAGHGAKNKLKPITILTKKSERFRKKLIERWVCEVAEFFIKNKVGTVQMENLESMKRKEDSYFNIRLRGFWPYAEMQNKIEFKLKQYGIEIRKVAPNNTSKTCSKCGHLNNYFNFEYRKKNKFPHFKCEKCNFKENADYNAALNISNPKLKSTKEEP

SEQ ID NO: 510 - protein, 726 aa, synthetic construct; identical to SEQ ID NO: 498

SEQ ID NO: 511 - protein, 726 aa, synthetic construct
SEVEFSHEYWMRHALTLAKRARDEREVPVGAILVLNNRVIGEGWNRAIGLHDPTAHAEIMALRQGGLVMQNYRLIDATLYVTFEPCVMCAGAMIHSRIGRVVFGVRNNKHGAAGSLVNVLNYPGMNHRVEITEGILADECAALLCDFYRMPRQVFNARKKAQSGINPGGSSGGSSGSGTPGTSESATPESSGGSSSGSAKNTITKTLKLRIVRPYNSAEVEKIVADEKNNREKIALEKNKDKVKEACSEHLKVAAYCTTQVGRNACLFCKARKLDDRFYQKLRGQFPDAVFWQEIGEIFRQLQKQAAEIYNQSLIELYYEIFIKGKGFANASSVEHYLSDVCYTRAAELFKNAAIASGLRGKVKSNFRLKELKNMKSSLPTTKSDNFPIPLVKQKGGQYTGFEISSHNDDFIIKIPFGRWQVKKEIDKYRPWEKFDFEQVRKSPKPISLLLSTQRRMRNKGWGKDEGTEAEIRKVMNGDYRTSYIEVKRGSKTGEKSAWMLNLSIDVPKIDKGVDPSIIGGIDVGVKSPLVCAINNAFSRYSISDNDLFRFNKKMFARRRILLRKNRHKRAGHGAKNKLKPISILTGKSERFRKKLIERWACEIADFFIKNKVGTVQMENLESMKRKEDSYFNIRLRGFWPYAEMQNKIEFKLKQYGIEIRKVAPNNTSKTCSKCGHLNNYFNFEYRKKNKFPHFKCEKCNFKENADYNAALNICNPKLKSTKEEP

SEQ ID NO: 512 - protein, 726 aa, synthetic construct
SEVEFSHEYWMSHALTLAKRARDEREVPVGAVLVLNNRVIGEGWNRAIGLHDPTAHAEIMALRQGGLVMQNYRLTDATLYVTFEPCVMCAGAMIHSRIGRVVFGVRNSKHGAAGSLVNVLNYPGMNHRVEITEGILADECAALLCDFYRMPRRVFNARMKAQSSISPGGSSGGSSGSDTPGTSESATPESSGGGSSGSAKNTITKTLQLRIVRPYNSAEVEKIVADEKNNREKIALEKNKDKVREACSKHLKVASYCTTQVERNACPFCKARKLDDKFYQKLRGQFPDAVFWQELGGIFRQLQKQAAEIYNQSLIELYYEIFIKGKGITNASRVEHYLSDVCYTRAAELFKNAAIASGLRGKVKSNFRLKELKNMKSGLPTTKSDNFPIPLVKQKGGQYTGFEISSHNDDFIIKIPFGRWQVKKEIDRYRPWEKFDFEQVRKSPKPISLLLSTRRRKRNKGWSKDEGTEAEIRKVMNGDYQTSYIEVKRGSKIGEKSAWMLNLSIDVPKIDKGVDPSIIGGIDVGVKSPLVCAINNAFGRYSISDNDLFHFNKKMFAMRRILLKKNRHKRAGHGAKNKLKPITILTEKSKRFRKKLIERWACEIADFFIKNKVGTVQMENLEGMKRKEDSYFNIRLRGFWPYAEMQNKIEFKLKQYGIEIRKVAPNNTSKTCSKCGHLNNYFNFEYRKKNKFPHFKCEKCSFKENADYNAALNICNPKLKSTKEEP

SEQ ID NO: 513 - protein, 726 aa, synthetic construct
SEVEFSHEYWMRHALTLAKRARDEREVPVGAVLVLNNRVIGEGWNRAIGLHDPTAHAEIMALRQGGLVMQNYRLTDATLYVTFEPCVMCAGAMIHSRIGRVVFGVRNSKRGAAGSLMNVLNYPGMNHCVEITEGILVDECAALLCDFYRMPRRVLNAQKKAQPSISSGGSSGGSGGNETPGASESVTPKSSGGGSAGSTKNTITKTLKLRIVRPYNSAEVEKIVADEKNSREKIALERNKDKVKEACSEHLKVAAYCTTQVERNACLFCKARKLDDRFYQKLRGQFPDAVFWQETGEIFRQLQRQAAEIYNRSLIELYYEIFIKGKGFANASSVEHYLSDVCYTRAAELFKNAAIASGLRGKVKSNFRLKELKNMKSGLPTTKSDNFPIPLVKQKGGQYAGFEISSHNDDFIIKIPFGRWQEKEEIDKYRPWEKFDFEQVRKSPKPISLLLSTQRRKRNKGWSKDEGTEAEIRKVMNGDYQTSYIEVKRGSKIGEKSAWMLSLSIDVPKIDKGVDPSTIGGIDVGVKSPLVCAINNAFCRYSISDNDLFHFNKKMFARRRILLKKSRHKRAGHGAKNKLKPISILTEKSKRFRKKLIERWACEIADFFIKNKVGTVQMENLESMKRKEDSYFNIRLRGFWPYAEMQNKIEFKLKQYGIKIRKVAPNNTSKTCSKCGHLNNYFSFEYRKKNKFPHFKCEKCNFKENADYNAALNISNPKLMSTKEEP

SEQ ID NO: 514 - protein, 726 aa, synthetic construct
SEVEFSHEYWMRHALTLAKRARDEREVPVGAVLVLNNRVIGEGWNRAIGLHDPTAHAEIMALRQGGLVMQNYRLIDATLYVTFEPCVMCAGAMIHSRIGRVVFGVRNNKHGAAGSLVNVLNYPGMNHRVEITEGILADECAALLCDFYRMPRQVFNARKKAQSSINPGGSSGGSSGSETPGTSESATPESSGSSSGSSAKNTITKTLKLRIVRPYNSAEVEKIVADEKNNRERIALEKNKDKVKEACSKHLKVAAYCTTQVERNACLFCKARRLDDKFYQKLRGQFPDAVFWQEIGEIFRQLQKQAAEIYNQSLVELYYEILIKGKGIANASSVEHYLSDVCYTRAAKLFKNAAIASGLRNKIKSNFRLKELKNMKSGLPTTKSDNFPIPLVKQKGGQYTGFEISSHNSDFIIKIPFGRWQEKEEIDKYRPWEKFDFEQVRKSPKPISLLLSTQRRKKNKGWGKDEGTEAEIRRVMNGNYQTSYIEVKRGSKIGEKSAWMLNLSIDVPKIDKGVDPSIIGGIDVGVKSPLVCAINNAFSRYSISDNDLFHFNKKMFARRRILLKKTRHKRAGHGAKNKLKPISILTEKSERFRKKLIERWACEIADFFVKNKVGTVQMENLESMKRREDSYFNIRLRGFWPYAKMLNKIEFKLKQYGIKIRKVAPNNTSKTCSKCGHLNNYFNFEYRKKNKFPHFKCEKCNFKENADYNAALNISNPKLKSTKGEP

SEQ ID NO: 515 - protein, 726 aa, synthetic construct
SEVEFSHEYWMRHALALAKRARDEREVPVGAVLVLNNRAIGEGWNRAIGLHDPTAHAEIMALRQGGLVMQNYRLTDATLYVTFEPCVMCAGAMIHSRIGRVVFGVRNSKRGAAGSLMNVLNYPGMNHCVEITEGILVDECAALLCDFYRMPRQVLNAQKKAQSTIYTGGSSGGSSGSEAPGTSESPTPESSGGSSGGSAKNTITKTLKLRIVRPYNSAEVEKIVADEKNNREKIALEKNKDKVKEACSKHLKVAAYCTTQVERNACLFCKARKLDDKFYQKLRGQFPDAVFWQEIGEIFRQLQKQAAEIYNQSLIELYYEIFIKGKGFANASSVEHYLSDVCYTRAAELFKNAAIASGLRGKVKSNFRLKELKNMKSGLPTTKSDNFPIPLVKQKGGQYTGFEISSHNDDFIIKIPFGRWQVKEEIDKYRPWEKFDFEQVRKSPKPISLLLSTRRRKRNKGWSKDVGTEAEIRKVMNGDYQTSYIEVKRGSKIGEKSAWMLNLSIDVPKIDKGVDPSIIGGIDVGVKSPLVCAINSAFSRYSISDNDLFRFNKKMFARRRILLKKNRHKRAGHGAKNKLKPITILTEKSRRFRKKLIERWACEIADFFIKNKVGTVQMESLESMKRKEDSYFNTRLRGFWPYAEMQNKIEFKLRQYGIKIRKVAPNNTSKTCSKCGHLNDYFNFEYRKKNKFPHFKCEKCNFKENADYNAALNISNPKLKSTKEEP

SEQ ID NO: 516 - protein, 726 aa, synthetic construct
SEVEFSHEYWMRHALTLAKRARDEREVPVGAVLVLNNRVIGVGWNRAIGLHDPTAHAEIMALRQGGLVMQNYRLIDATLYVTFEPCIMCAGAMIHSRIGRVVFGVRNNKHGAAGSLVNVLNYPGMNHRVEITEGILADECAALLCDFYRMPRQVFNARKKAQSSINPGGSSGGSSGSETPGTSESATPESSGGSSGSSAKNTITKTLKLRIVRPYNSAEVEKIVADEKNNREKIALEKNKDKVKEACSKHLKVAAYCTTQVERNACLFCKARRLDDKFYQKLRGQFPDAVFWQEIGEIFRQLQKQAAEIYNQSLVELYYEIFIKGKGIANASSVEHYLSDVCYTRAAELFKNAAIASGLRNKIKSNFRLKELRNMKSGLPTTKSDNFPIPLVRQKGGQYTGFEISNHNGDFIIKIPFGRWQVKKEICKHRPWEKFDFEQVRKSPKPISLLLSTQRRKRNKGWGKDEGTEAEIRKVMNGDYQTSYIEVKRGSKIGEKSAWMLNLSIDVPKIDKGVDPSIIGGIDVGVKSPLVCAINNALSRYSISDNDLFHFNKKMFARRRILLRKNRHKRAGHGAKNKLKPITILTEKSGRFRKKLIERWACEIADFFIKNKVGTVQMENLESMKRREDSYFNIRLRGFWPYAEMQNKIEFKLKQYGIEIRKVAPNNTSKTCSKCGHLNDYFNFEYRKKNKFPHFKCEKCNFKENADYNAALNISNPKLKSTKEEP

SEQ ID NO: 517 - protein, 726 aa, synthetic construct
SEVEFSHEYWMRHALTLAKRARDEREVPVGAILVLNNRVIGEGWNRAIGLNDPTAHAEIMALRQGGLVMQNYRLIDATLYVTFEPCVMCAGAMVHSRIGRVVFGVRNSKRGAAGSLMNVLNYPGVNHCVEITEGILVDECAALLCDFYRMPRQVLNAQKKAQSSISSGGSSGGCSGSEMPGASESVTPKSSGGSSAGSTKNAITKTLKLRIVRPYNSAEVEKIVADEKNSREKIALEKNKDKVKEACSEHLKVAAYCTTQVERNACLFCKARKLDDRFYQKLRGQFPDAVFWQETGEIFRQLQRQAAEIYNQSLIELYYEIFIKGKGFANASSVEHYLSDVCYTRAAELFKNAAIASGLRGKVKSNFRLKELKNMKSGLPTTKSDNFPIPLVKQKGGQYTGFEISSHNDDFIIKIPFGRWQVKEEIDKYRPWEKFDFEQVRRNPKPISLLLSTQRRKRNKGWSKDEGTEAEIRKVMNGDYQTSYIEVKRGSKVGEKSAWMLNLSIDVPKIDKGVDPSIIGGIDVGVKSPLVCAINNAFSRYSISDNDLYRFNKKMFARRRILLKKSKHKRAGHGAKNKLKPITILTEKSGRFRKKLIERWACEIADFFIKNKVGTVQMENLEGMKRKEDSYFNIRLRGFWPYAEMQNKIEFKLKQYGIVVRKVAPNNTSKTCSKCGHLNNYFNFEYRKKNKFPHFKCEKCNFKENADYNAALNISNPVLKSTKGEP

SEQ ID NO: 518 - protein, 726 aa, synthetic construct
SEVEFSHEYWMRRALTLARRARDEREVPVGAVLVLNSRVIGVGWNRAVSLHDPTAHAEIMALRQGGLVMQNHRLIDATLYVTFEPCVMCAGAMVHSRIGRVVFGVRNSKRGAAGSLMNVLNYPGMNHRVEITEGVLADECAALLCDFYRMPRQVLNAQRKAQSSINFGGPSGGSSGSGTPGTSESAAPESSGGSSGGSAKNTITKTLKLRIVRPYNSAEVEKIVADEKNNRERIALEKNKDKVREACSKHLKVASYCTTQVERNACPFCKARKLDDKFYQKLRGQFPDAVFWQELGEIFRQLQKQAAEIYNQSLIELYYEIFIKGKGFANASSVEHYLSDVCYARAAELFKNAAIASGLRGKVKSNFRLKELKNMKSGLPTTKSDNFPIPLVKQKGGQYTGFEISSHNDDFIIKIPFGRWQVKKEIDKYRPWEKFDFEQVRKSPKPISLLLSTQRRKRNKGWSKDEGTEAEIRKVMNGDYQTSYIEVKRGSKTGEKSTWMLNLSIDVPKIDKGVDPSIIGGIDVGVKSPLVCAINNAFSRYSISDNDLFRFNKKMFARRRILLKKNRHKRAGHGAKNKLKPISILTGKSERFRKKLIERWACEIADFFIKNKVGTVQMENLESMKRKEDSYFNIRLRGFWPYAEMQNKIEFKLKQYGIKIRKVAPNNTSKTCSKCGHLNNYFSFEYRKKNKFPHFKCEKCNFKGDADYNAALNISNPKLKSTKEEP

SEQ ID NO: 519 - protein, 726 aa, synthetic construct
SEVEFSHEYWMRHALTLAKRARDEREVPVGAVLVLNNRVIGEGWNRAIGLHDPTAHAEIMALRQGGLVTQNYRLIDATLYVTFEPCVMCAGAMIHSRIGRVVFGVRNSKHGAAGSLMNVLNYPGMNHHVEITEGILVDECAALLCDFYRMPRQVFNARKKAQSSINPGGSFGGSSGSETPGTSESATLESSGGSSGGSAKNTITKTLKLRIVRPYNSAEVEKIVADEKDNREKIALEKNKDKVKEACSKHLKVAAYCTTQVERNACQFCKARKLDDKFYQKLRGQFPDAVFWQEIGEIFRQLQKQAAEIYNQSLIELYYEIFIKGKGFANASSAEHYLSDVCYTRAAELFKNAAIASGLRGKVKSNFRLKELKNMRSGLPTTKSDNFPIPLVKQKGGKYTGFEISSHNDDFIIKIPFGRWQVKKVIDKYRPWEKFDFEQVRKSPKPISLLLSTQRRKRNKGWSKDEGTEAEIRKVMNGDYQTSYIEVKRGSKIGEKSAWMLNLSIDVPKIDKGVDPSIIGGIDVGVKSPLVCAINNAFSRYSISDNDLFHFNKKMFARRRILLKKNRHKRAGHGAKNKLKPISILTEKSKRFRKKLIERWACEIADFFIKNKVGTVQMENLESMKRKEDSYFNIRLRGFWPYAEMQNKIEFKLKQYGIEIRKVAPNNTSKTCSKCGHLNYYFNFEYRKKNKFPHFKCEKCNFKEDADYNAALNISNPKLKSTKEEP

SEQ ID NO: 520 - protein, 726 aa, synthetic construct
SEVEFSHEYWMRHALTLARRARDGREVPVGAVLVLNNRVIGEGWNRAIGLHDPTAHAEIMALRQGGLVMQNYRLIDATLYVTFEPCVMCAGAMVHSRIGRVVFGVRNSKRGAAGSLMNVLDYPGMDHRVEITEGILADECAALLCDFYRMPRQVFNAQKKAQSSINSGGSSGGSSGSETPGTSESATPESSGGSSGGSAKNTITKTLQLRIVRPYNSAEVEKIVTDEKNNREKIALEKNKDKVKEACSKHLKVATYCTTQVERNACLFCKARKLDDKFYQKLRGQFPDAVFWQEIGEIFRQLQKQAAEIYNQSLIELYYEIFIEGKGSANARSVEHYLSDVCYTRAAELFKNAAIASGLRGKVKSNFRLKELKNMKSGLPTTKSDNFPIPLVKQKGGQYTGFEISSHNDDFIIKIPFGRWQVKEEIDKYRPWEKFDFEQVRKSPKPISLLLSTQRRKRNKGWGKDEGTEAEIRKVMNGDYQTSYIEVKRGSKIGEKSAWMLSLSIDVPKIDKGVDPRIIGGIDVGVKSPLVCAINNAFSRYSISDNDLFHFNKKMFARRRILLRKNRHKRAGHGAKNKLKPITIMTEKSKRFRKKLIERWACEIADFFIKNKVGTVQMENLESMKRKEDSYFNIRLRGFWPYAEMQNKIEFKLRQYGIVVRKVAPNNTSKTCSKCGHLNNYFDFEYRKKNKFPHFKCEKCNFKENADYNAALNISNPKLKSTKEEP

SEQ ID NO: 521 - protein, 726 aa, synthetic construct
SEVEFSHEYWMRRALTLAKRARDEREVPVGAVLVLNNRVIGEGWNRAIGLHDPTAHAEIMALRQGGLVMQNHRLVDATLYVTFEPCVLCAGAMVHSRIGRVVFGVRNSKRGAAGSLMNVLNYPGMNHRVEITEGILADECAALLCDFYRMPRQVFNAQKKARSNINSGGSSGGSSGSETPGTSESATPESSGGGSSGSAKNTITKTLQLRIVRPYNSAEVEKIVADEKNNREKIALEKNKDKVKEACSKHLKVASYCTTQVERNACPFCKARKLDDKFYQKLRGQFPDAVFWQELGEILRQLQKQAAEIYNQSLIELYYEIFIKGKGITNASRVEHYLSDVCYTRAAELFKNAAIASGLRSKVRSNFRLKELKNMKSGLPTTKSDNFPIPLVKQKGGQYTGFEISSHNDDFIIKIPFGRWQVKEEIDKYRPWEKFDFEQVRKNPKPISLLLSTQRRKRNKGWSKDEGTEAEIRKVMNGDYQTSYIEVKRGSKIGEKSAWMLNLSIDVPKIDKGVDPSIIGGIDVGVKSPLVCAINNAFSRYSVSDNDLFRFNKKMFARRRILLKKNRHKRAGHGAKNKLKPISILTEKSKRFRKKLIERWACEIADFFIKNKVGTVQMENLESMKRKEDSYFNIRLRGFWPYAEMQNKIEFKLKQYGIEIRKVAPNNTSKTCSRCGHQNNYFNFEYRRRNKFPHFKCEKCNFKENADYNAALNISNPKLKSTKEEP

SEQ ID NO: 522 - protein, 726 aa, synthetic construct
SEVEFSHEYWMRYALTLAKRARDEREVPVGAVLVLNNRVIGEGWNRAIGLHDPTAHAEIMALRQGGLVMQNYRLIDATLYVTFEPCVMCAGAMIHSRIGRVVFGVRNSKRGAAGSLMNVLNYPGMNHRVEITEGILADECAALLCDFYRMPRQVLNAQKRARSCINSGGSSGGSSGSETPGTSESATPETPGGSSGGSAKNTITKTLKLRIVRPYNSAEVEKIVADEKDNRERIALEKNKGKVKEACSKHLKVAAYCTTQVERNACLFCKARKLDDKFYQKLRGQFPDAVFWQELGEILRQLQKQAAEIYNQSLIELYYEIFIKGKGFANASSVEHYLSDVCYTRAAELFKNAAIASGLRGKVKSNFRLKELKNMKSGLPTTKSDNFPIPLVKQKGGQYTGFEISNHNSDFIIKIPFGRWQAKKEIDKYRPWEKFDFEQVRKSPKPISLLLSTQRRKRNRGWSKDEGTEAEIRKVMNGDYQTSYIEVKRGSKTGEKSAWVLNLSIDVPKIDKGVDPSIIGGIDVGVKSPLVCAINNAFSRYSISDNDLFRFNKKMFARRRILLKKNRRKRAGHGAKNKLKPISILTEKSERFRKKLIERWACEIADFFIKNKVGTVQMENLESMKRREDSYFNIRLRGFWPYAEMQNKIEFKLKQYGIKVRKVAPNNTSKTCSKCGHLNNYFSFEYRKKNKFPHFKCEKCNFKENADYNAALNISNPKLKSTKEEP

SEQ ID NO: 523 - protein, 726 aa, synthetic construct
SEDEFSHEYWMRHALTLARRARDGREVPVGAVLVLNNRVIGEGWNRAIGLHDPTAHAEIMALRQGGLVMQNYRLIDATLYVTFEPCVMCAGAMVHSRIGRVVFGVRNSKRGAAGSLMNVLDYPGMGHRVEITEGILADECAALLCDFYCMPRQVFNAQKRAQSSINSGGSSGGSSGSETPDTSESATPESSGGGSSGSAKNTITKTLQLRIVRPYNSAEVEKIVADEKNNREKIALEKNKDKVKEACSKHLKVASYCTTQVERNACPFCKARKLDDKFYQKLRGQFPDAVFWQELGEILRQLQKQAAEIYNQSLIELYYEIFIKGRGFANASSVEHYLSDVCYTRAAELFKNAAIASGLRGKVKSNFRLKELKNMKSGLPTTKSDNFPIPLVKQKGGQYTGFEISSHNDDFIIKIPFGRWQAKKEIDKYRPWEKFDFEQVRKSPKPISLLLSTQRRKRNKGWSKDEGTEAEIRKVMNGDYQTSYIEVKRGSKTGEKSAWMLNLSIDVPKIDKGVDPSIIGGIDVGVKSPLVCAINNAFSRYSISDNDLFRFNKKMFARRRILLKKNRHKRAGHGAKNKLKPISILTEKSKRFRKKLIERWACEIADFFIKNKVGTVQMENLESMKRKEDSYFNIRLRGFWPYAEMQNKIEFKLKQYGIEIRKVAPNNTSKTCSKCGHLNNYFNFEYRKMNKFPHFKCEKCNFKENADYNAALNISNPKLKSTKEEP

SEQ ID NO: 524 - protein, 726 aa, synthetic construct
SEVEFSHEYWMRHALTLAKRARDEREVPVGAVLVLNNRVIGEGWNRAIGLHDPTAHAEIMALRQGGLVMQNYRLVDATLYVTFEPCVLCAGAMVHSRIGRVVFGVRNSKRGAAGSLMNVLNYPGMNHRVEITEGILADECAALLCDFYRMPRQVFNAQKKARSNINSGGSSGGSSGSETPGTSESATPVSSSGSSGGSAKNTITKTLQLRIVRPYNSAEVEKIVADEKNNREKIALEKNKDKVKEACSKHLKVASYCTSQVERNACPFCKARKLDDKFYQRLRGQFPDAVFWQELGEILRQLQKQAAEIYNQSLIELYYEIFIKGRGFANASSVEHYLSDVCYTRAAELFKNAAIASGLRGKVKSNFRLKELKNMKSGLPTTKSDNFPIPLVKQKGGQYTGFEISNRNSDFIIKIPFGRWQVKKEINKYRPWEKFDFEQVRKSPKPISLLLSTQRRKRNKGWSKDEGTEAEIRKVMNGDYQTSYIEVKRGSRIGEKSAWMLSLSIDVPKIDRGVDPSIIGGIDVGVKSPLVCAINNALSRYSISDNDLFHFNKKMFARRRILLKKNRHRRAGHGARNKLKPITVLTEKSKRFRKKLIERWACEIANFFIKNKVGTVQMENLESMKRKEDSYFNIRLRGLWPYAEMQNKIEFKLKQYGIEIRKVAPNNTSKTCSKCGHLNNYFNFEYRKRNKFPHFKCEKCNFKENADYNAALNISNPKLKGTKEEP

SEQ ID NO: 525 - protein, 726 aa, synthetic construct
SEVEFSHEYWMRHALTLAKRARDEREVPVGAVLVLNNRVIGEGWNRAIGLHDPTAHAEIMALRQGGLAMQNYRLVDATLYVTFEPCVLCAGAMVHSRIGRVVFGVRNSKRGAAGSLMNVLNHPGMNHRVEITGGILADECAALLCDFYRMPRQVFNAQKKARSNINSGGSSGGSSGSETLGTSESATPESSGGSSGGSAKNTITKTLKLRIVRPYNSAEVEKIVADEKNNREKTALEKNKDKVKEACSKHLKVAAYCTTQVERNACLFCKARKLDDKFYQKLRGQFPDAVFWQEVGEIFRQLQKQAAEIYNQSLIELYYEIFIKGKGFANASSVEHYLSDVCYTRAAELFKNAAIASGLRGKVKSNFRLKELKNMKSGLPTTKSDNFPIPLVKQKGGQYTGFEISNRNSDFIIKIPFGRWQVKKEINKYRPWEKFDFEQVRKSPKPISLLLSTQRRKRNKGWSKDEGTEAEIRKVMNGDYQTSYIEVKRGSRIGEKSAWMLSLTVDVPKIDRGVDPSIIGGIDVGVKSPLVCAINNALSRYSISDNDLFHFNKKMFARRRILLKKNRHRRAGHGARNKLKPITVLTEKSMRFRKKLIERWACEIANFFIRNKVGTVQMENLESMKRKEDSYFNIRLRGLWPYAEMQNKIEFKLKQYGIEIRKVAPNNTSRTCSKCGHLNNYFNFEYRKKNKFPRFKCEKCNFKENADYNAALNISNPRLKSTKEEP

SEQ ID NO: 526 - protein, 726 aa, synthetic construct
SEVEFSHEYWMRHALILAKRARDEREVPVGAVLVLNNRVIGEGWNRAIGLHDPTAHAEIMALRQGGLVMQNYRLSDATLYVTFEPCVMCAGAMIHSRIGRVVFGARNSKRGAAGSLMNVLNYPGMNYCVEITEGILVDECAALLCDFYRMPRQVLSAQKKAQSSISSGGLSGGSSGSETPGTSGGVTPKSSVGSSAGSTKNTITKTLKLRIVRPYNSAEVEKIVADEKNNREKIALEKNKDKVKEACSKHLKVAAYCTTQVERNACLFCKARKLDDKFYQKLRGQFPDAVFWQEIGEIFRQLQKQAAEIYNQSLIELYYEIFIKGKGFANASSVEHYLSDVCYTRAAELFKNAAIASGLRGKVKSNFRLKELKNMKSGLPTTKSDNFPIPLVKQKGGQYTGFEIRSHNDDFVIKIPFGRWQVKKEIDKYRPWEKFDFEQVRKSPKPISLLLSTQRRKRNKGWSKDEGTEAEIRKVMNGDYQTSYIEVKRGSKIGEKSAWMLNLSIDVPKIDKGVDPSIIGGIDVGVKSPLVCAINNAFSRYSISDNDLFHFNKKMFARRRILLKKSKHKRAGHGAKNKLKPITIMTEKSKRFRKKLIERWACEIADFFIKNKVGTVQMENLESMKRREDSYFNIRLRGFWPYAEMQNKIEFKLKQYGIVVRKVAPNNTSKTCSKCGHLNNYFNFEYRKKNKFPHFKCEKCNFKEDADYNAALNISNPKLKSTKGEP

SEQ ID NO: 527 - protein, 726 aa, synthetic construct
SEVEFSHEYWMRHALTLAKRARDEREVPVGAVLVLNNRVIGEGWNRAIGLHDPTAHAEIMALRQGGLVMQNYRLTDATLYVTFEPCVMCAGAMIHSRIGRVVFGIRNSKRGAAGSLMNVLNYPGMNHCVEITEGILVDECAALLCDFYRMPRQVLNAQKRAQSSISSGGSSGGSSGSETPGTSESATPGSSGGSSGGSAKNTITKTLKLRIVRPYNSAEVEKIVADEKNYREKIALEKNKDKVKEACSEHLKVAAYCTTQVERNACLFCKARKLDDKFYQKLRGQFPDAVFWQEIGEIFRQLQKQAAEIYNQSLIELYYEILIKGKGFANASSVEHYLSDVCYTRAAELFKNAAIASGLRGKVKSNFRLKELKNMKSGLPTTKSDNFPIPLVKQKGGQYTGFEISSHNDDFIIKIPFGRWQAKKEIDKYRPWEKFDFEQVRKSPKPISLLLSTQRRKRNRGWSKDEGTEAEIRKVMNGDYQTSYIEVKRGSKIGEKSAWMLNLSIDVPKIDKGVDPSIIGGIDVGVKSPLVCAVNNAFSRYSISDNDLFRFNKKMFARRRILLGKNRHKRAGHGTKNKLKPITILTEKSGRFRKKLIERWACEIANFFIKNKVGTVQMENLESMKRKEDSYFNIRLRGFWPYAEMQNKIEFKLKQYGIEIRKVAPNNTSKTCSKCGHLNNYFSFEYRKKNKFPHFKCEKCNFKEDADYNAALNISNPKLKSTKEEP

SEQ ID NO: 528 - protein, 726 aa, synthetic construct
SEVEFSHEYWMRHALMLAKRARDEREVPVGAVLVLNNRVIGEGWNRAIGLHDPTAHAEIMALRQGGLVMQNYRLTDATLYVTFEPCVMCAGAMIHSRIGRVVFGVRNSKRGAAGSLMNVLSYPGMNHCVEITEGILVDECAALLCDFYRMPRRVLNAQKKAQSSISSGGPSGGSSGSETPGTSESATPESSGGSSGGSAKNTITKTLKLRIVRPYNSTEVEKIVADEKNNREKIALEKNKDKVKEACSKHLKVASYCTTQVERNACLFCKARKLDDKFYQKLRGQFPDAVFWQELGEIFRQLQKQAAEVYNQSLIELYYEIFIKGKGFANASSVEHYLSDVCYTRAAELFKNAAIASGLRGKVKGNFRLKELRSMKSGLPTTKSDNFPIPLVRQKGGQYTGFEISSHNDDFIIKIPFGRWQVKREIDKYRPWEKFDFEQVRKSPKPISLLLSTQRRKRNKGWSKDEGTEAEIRKVMNGDYQTSYIEVKRGSKIGEKSAWMLNLSIDVPKIDKGVDPSIIGGIDVGVKSPLVCAINNAFSRFSISDNDLFHFNKKMFARRRILLKKNRHRRAGHGVKNKLKPITILAEKSKRFRKKLIERWACEIADFFVKNKVGTVQMENLESMKRKEDSYFNIRLRGFWPYAEMQNKIEFKLKQYGIEIRKVAPNNTSRTCSKCGHLNNYFNFEYRKKNKFPHFKCEKCNFKENADYNAALNISNPKLKSTKEEP

SEQ ID NO: 529 - protein, 726 aa, synthetic construct
SEVEFSHEYWMRHALTLAKRARDEREVPVGAVLVLNNRVIGEGWNRAIGLHDPTAHAEIMALRQGGLAMQNYRLVDATLYVTFEPCVLCAGAMVHSRIGHVVFGVRNNKRGAAGSLMNVLNYPGMNHRVEITEGILADECAALLCDFYRMPRRVFNAQKKARSNTNSGGSSGGSSGSETPGTSEGATPESSGGSSGGSAKNTITKTLKLRIVRPYNSAEVEKIVADEKNNREKIALEKNKDKVKEACSKHLKVASYCTTQVERNACLFCKARKLDDKFYQKLRGQFPDAVFWQELGEIFRQLQKQAAEIYNQSLIELYYEIFIKGKGFANASSVEHYLSDVCYTRAAELFKNAAIASGLRGKVKSNFRLKELRNMKSGLPTTKSDNFPIPLVKQKGGQYTGFEISSHNDDFIIKIPFGRWQMKKEIDRYRPWEKFDFEQVRKSPKPISLLLSTQRRKRNKGWSKDEGTEAEIRKVMNGDYQTSYIEVKRGSKIGEKSAWMLNLSIDVPKVDKGVDPSIIGGIDVGVRSPLVCAINNAFSRYSISDNDLFHFNKKMFARRRILLKKNRHRRAGHGAKNKLKPIAVLAEKSEGFRKKLIERWACEVADFFIKNKVGTVQMENLESMKRREDSYFNIRLRGFWPYAEMQNKIEFKLRQYGIEIRKVAPNNTSKTCSKCGHLNNYFNFEYRKKNKFPHFKCEKCNFKENADYNAALNISNPKLKSTKEKP

SEQ ID NO: 530 - protein, 726 aa, synthetic construct
SEVEFSHEYWMRHALTLAKRARDEREVPVGAVLVLNNRVIGEGWNRAIGLHDPTAHAEIMALRQGGLVLQNYRLVDATLYVTFEPCVLCAGAMVHSRIGRVVFGARNSKRGAAGSLMNILNYPGMNHRVEITEGILADECAALLCDFYRMPRQVFNAQKKAQSSINSGGSSGGSSGSETPSTSESATPESSGGSSGGSAKNTITKTLQLRIVRPYNSAEVEEIVTDEKNNREKIALEKNKDKVKEACSKHLKMASYCTTQVERNACLFCKARELDDKFYQKLRGQFPDAVFWQELGGIFRQLQKQAAEIYNQSLIELYYEIFIKGKGITNASRVEHYLSDVCYTRAAELFKNAAIASGLRSKVRSNFRLKELKNMKSGLPTTKSDNFPIPLVKQKGGQYTGFEISSHNSDFIIKIPFGRWQVKEEIDKFRPWEKFDFEQVRKSPKPISLLLSTQRRKKNKGWSKDEGTEAEIRKVMNGDYQTSYIEVKRGSKTGEKSAWMLNLSIDVPKIDKGVDPSIIGGIDVGVKSPLVCAINNAFSRYSISDNDLFRFNKKMFARRRILLKKNRHKRAGHGTKNKLKPITTLTEKSGRFRKKLIERWACEIANFFIKNKVGTVQMENLESMKRKEDSYFNIRLRGFWPYAEMQNKIEFKLKQYGIKIRKVAPNNTSKTCSKCGHLNNYFSFEYRKKNKFPHFKCEKCNFKEDADYNAALNISNPKLKSTKEEP

SEQ ID NO: 531 - protein, 726 aa, synthetic construct
SEVEFSHEYWMRHALTLAKRARDEREVPVGAILVLNNRVIGVGWNRAIGLHDPTAHAEVMALRQGGLVTQNYRLIDATLYVTFEPCVMCAGAMIHSRIGRVVFGVRNSKHGAAGSLVNVLNYPGMNHRVEITEGILADECAALLCDFYRMPRQVFNARKKAQSSINSGGSSGGSSGSETPGTSESATPKSSGGSSGGSAKNTITKALKLRIVRPYNSAEVEKIVADEKNNRERIALEKNKDKVKEACSKHLKVAAYCTTQVERNACLFCKARKLDDKFYQKLRGQFPDAVFWQEIGEIFRQLQKQAAVIYNQSLIELYYEIFIKGKGFANASSVEHYLSDVCYTRAAELFKNAAIASGLRGKVKSNFRLKELKNMKSGLPTTKSDNFPIPLVKQKGGQYTGFEISSHNDDFIIKIPFGRWQVKKEIDKYRPWEKFDFEQVRKSPKPISLLLSTRRRKRNKGWSKDEGTEAEIRKVMNGDYQTSYIEVKRGSKIGEKSAWMLNLSIDVPKIDKGVDPSIIGGIDVGVKSPLVCAINNALSRYSISDNDLFHFNKKMFARRRILLRKNRHKRAGHGAKNKLKPITIMTEKSKRFRKKLIERWACEIADFFIKNKVGTVQMENLESMKRKEDSYFNIRLRGFWPYAEMQSKIEFKLKQYGIVVRKVAPNNTSKTCSKCGHLNNYFNFEYRKKNKFPHFKCEKCNFKEDADYNAALNISNPKLKSTKGEP

SEQ ID NO: 532 - protein, 726 aa, synthetic construct
SEVEFSHEYWMRHALTLAKRARDEREVPVGAVLVLNNRVIGEGWNRAIGLHDPTAHAEIMALRQGGLAMQNYRLVDATLYVTFEPCVLCAGAMVHSRIGRVVFGVRNSKRGAAGSLMNVLNYPGMNHRVEITEGILADECAALLCDFYRMPRQIFNARKKARSNTNSSGSSGGSSGSETTGTSESATPESSGGSSGGSAKNTITKTLKLRIVRPYNSAEVEKIVADEKNSREKIALEKNKDKVREACSRHLKVASYCTTQVERNACPFCRARKLDDKFYQKLRGQFPDAVFWQELGEILRQLQKQAAEIYNQSLIELYYEIFIKGRGFANASSVEHYLSDVCYTRAAELFKNAAIASGLRGKVKSNFRLKELKNMKSGLPTTKSDNFPIPLVKQKGGQYTGFEISSHNDDFIIKIPFGRWQVKKEIDKYRPWEKFDFEQVRKSPKPISLLLSTQRRKRNKGWSKDEGTEAEIRKVMNGDYRTSYIEVKRGSKTGEKSAWMLNLSIDVPKIDKGVDPSIIGGIDVGVKSPLVCAINNAFSRYSISDNDLFHFNKKVFARRRILLKKNRHKRAGHGAKNKLKPITILTEKSKRFRKKLIERWACEIADFFIKNKVGTVQMENLESMKRKEDSYFNIRLRGFWPYAEMQDKIEFKLKQYGIEIRKVAPNNTSKTCSRCGHLNNYFNFEYRRKNKFPHFKCEKCNFKENADYNAALNISNPKLKSTKEEP

SEQ ID NO: 533 - protein, 726 aa, synthetic construct
SEVEFSHEYWMRHALTLAKRARDEREVPVGAVLVLNNRVIGEGWNRAIGLHDPTAHAEIMALRQGGLVMQNYRLVDATLYVTFEPCVMCAGAMIHSRIGRVVFGIRNNKHGAAGSLMNVLNYPGMNHRVEITEGILADECAALLCDFYRMPRQVFNARKKAQSSINPGGPSGGNSGSKTPGTSESATSEGSGGSSGGSAKNTITKTLKLRIVRPYNSAEVEKIVADEKNNREKIALEKNKDKVKEACSKHLKVASYCTTQVERNACLFCKARKLDDKFYRKLRDQFPDAVFWQEVGEIFRQLQKQAAEVYNQSLVELYYEILIKGKGIANASSVEHYLSDVCYTRAAELFKNAAIASGLRNKIKSNFRLKELRNMKSGLPTTKSDNFPIPLVRQKGGQYTGFEISSHNDDFIIKIPFGRWQVKKETNKYRPWEKFDFEQVRKSPKPISLLLSTQRRMRNKGWSKDEGTEAEIRKVMNGDYQTSYIEVKRGSKIGEKSAWMLNLSIDVPKIDKGVDPSIIGGIDVGVKSPLVCAINNALSRYSISDNDLFHFNKKMFARRRILLKKNRHKRAGHGARNKLKPITVLTEKSERFRKKLIERWACEIANFFIKNKVGTVQMENLESMKRKEDSYFNIRLRGFWPYAEMQNKIEFKLKQYGIEIRKVAPNNTSKTCSKCGHLNNYFNFEYRKTNKFPYFKCEKCNFKEDADYNAALNISNPKLKSTKEEP

SEQ ID NO: 534 - protein, 726 aa, synthetic construct
SEDEFSHEYWMRHALTLAKRARDGREVPVGAVLVLNNRVIGEGWNRAIGLHDPTAHAEIMALRQGGLVMQSYRLIDATLYVTFEPCVMCAGAMVHSRIGRVVFGVRNSKRGAAGSLMNVLDCPGMGHRVEITEGILADECAALLCDFYCMPRQVFNAQKRAQSSINSGGSSGGSSGSETPGTSESATPESSGGGSSGSAKNTITKTLQLRIVRPYNSAEVEKIVADEKNNREKIALEKNKDKVKEACSEHLKVASYCTTQVERNACLFCKARKLDDKFYQKLRGQFPDAVFWQELGGIFRQLQKQAAEIYNQSLIELYYEIFIKGKGITNASRVEHYLSDVCYTRAAELFKNAAIASGLRSKVRSNFRLKELKNMKSGLPTTKSDNFPIPLVKQKGGQYTGFEISSHNSDFIIKIPFGRWQVKEEIDKYRPWEKFDFEQVRKSPKPISLLLSTQRRKKNKGWSKDEGTEAEIRRVMNGDYRTSYIEVKRGSKIGEKSAWMLNLSIDVPKIDKGVDPSIIGGIDVGVKSPLVCAINNSSSRYSICDNDLFRFNKKMFARRRILLKKNRHKRAGHGAKNKLKPITILTKKSERFRKKLIERWVCEVADFFIKNKVGTVQMENLESMKRREDSYFNIRLRGFWPYAEMQSKIEFKLKQYGIEIRKVAPNNTSKTCSKCGHLNNYFSFEYRKKNKFPHFKCEKCNFREDADYNAALNISNPKLKSTKEEP

SEQ ID NO: 535 - protein, 726 aa, synthetic construct
SEVEFSHEYWMRHALTLAKRARDEREVPVGAILVLNNRVIGEGWNRAIGLHDPTAHAEIMALRQGGLVTQNYRLIDATLYVTFEPCVMCAGAMIHSRIGRVVFGVRNSKHGAAGSLMNVLNYPGMNHRVEITEGVLADECAALLSDFYRMPRQVFNAQKKARPYINSGGSSGGSSGSETPGTSESPTPESSGGSSGGSAKNTITKTLKLRIVRPYNSAEVEKIVADEKNNREKIALEKNKDKVKEACSKHLKVAAYCTTQVERNACLFCKARKLDDKFYQKLRGQFPDAVFWQEIGEIFRQLQKQAAEIYNQSLVELYYEIFIKGKGFANASSVEHYLSDVCYTRAAELFKNAAIASGLRGKVKGNFRLKELKSMKSGLPTTKSDNFPIPLVKQKGGQYTGFEISSHNDDFIIKIPFGRWQVKKEIDKYRPWEKFDFEQVRKSPKPISLLLSTQRRKRNKGWSKDEGTEAEIRKVMNGDYQTSYIEVKRGSKIGEKSAWMLSLSIDVPKIDKGVDPSIIGGIDVGVKSPLVCAINNAFCRYSISDNDLFHFNKKMFARRRILLKKSRHKRAGHGAKNKLKPISILTDKSKRFRKKLIERWACEIADFFIKNKVGTVQMENLESMKKKEDSYFNIRLRGFWPYAEMQNRIEFKLKQYGIEIRKVAPNNTSKTCSKCGHLNNYFNFEYRKKNKFPHFKCEKCNFKENADYNAALNISNPKLKSTKEEP

SEQ ID NO: 536 - protein, 726 aa, synthetic construct
SEVEFSHEYWMRHALTLAKRARDEREVPVGAVLVLNNRVIGEGWNRAIGLHDPTAHAEIMALRQGGLVMQNYRLTDATLYVTFEPCVMCAGAMIHSRIGRVVFGVRNSKRGAAGSLMNVLNYPGMNHRVEITEGILVDECAALLCDFYRMPCQVLNAQKKAQSSISSGGSSGGSSGGDTLGASESVTPKSSVGSSASSTKNTITKTLKLRIVRPYNSAEVEKIVADEKSNREKIALEKNKDKVKEACSKHLKVASYCTTQVERNACPFCKARKLDDKFYQKLRGQFPDAVFWQEIGEIFRQLQKQAAEIYNQSLIELYYEIFIKGKGFANASSVEHYLSDVCYTRAAELFKNAAIASGLRGKVKSNFRLKELKNMKSGLPTTKSDNFPIPLVKQKGGQYTGFEISSHNDDFIIKIPFGRWQVKEEIDKYRPWEKFDFEQVRKNPKPISLLLSTQRRKRNKGWSKDEGTEAEIRKVMNGDYQTSYIEVKRGSKIGEKSAWMLNLSIDVPKIDKGVDPSIIGGIDVGVKSPLVCAVNNAFSRYSISDNDLFRFNKKVFARRRILLKKNRHKRAGHGAKNKLKPITILTEKSGRFRKKLIERWACEIADFFIKNKVGTVQMENLESMKRKEDSYFNIRLRGFWPYAEMQNKIELKLKQYGIKIRKVAPNNTSKTCGKCGHLNDYFNFEYRKKNKFPHFKCEKCNFKEDADYNAALNISNPKLKSTKGEP

SEQ ID NO: 537 - protein, 726 aa, synthetic construct
SEVEFSHEYWMRHALTLAKRARDEREVPVGAILVLNNRVIGEGWNRAIGLHDPTAHAEIMALRQGGLVMQNYRLIDATLYVTFEPCVMCAGAMIHSRIGRVVFGVRNNKHGAAGSLVNVLNYPGMNHRVEITEGILADECAALLCDFYRMPRQVFNARKKAQSSINSGGSSGGSSGSETPGTSESATPKSSGGSSGGSAKNTITKALKLRIVRPYNSAEVEKIVADEKNNRERIALEKNKDKVKEACSKHLKVAAYCTTQVERNACLFCKARKLDDKFYQKLRGQFPDAVFWQEIGEIFRQLQKQAAEIYNQSLIELYYEIFIKGKGFANASSVEHYLSDVCYTRAAELFKNAAIASGLRGKVKSNFRLKELKNMRSGLPTTKSDNFPIPLVKQKGGQYAGFEISSHNDDFIIKIPFGRWQVKKEIDKYRPWEKFDFEQVRKSPKPISLLLSTQRRKRNKGWSKDEGTEAEIRKVMNGDYQTSYIEVKRGSKTGEKSAWMLNLSIDVPKIDKGVDPSIIGGIDVGVKSPLVCAINNAFSRYSISDNDLFHFNKKMFARRRILLKKTRHKRAGHGAKNKLKPISILTEKSERFRKKLIERWACEIADFFVKNKVGTVQMENLESMKRREDSYFNIRLRGFWPYAKMQNKIEFKLKQYGIEIRKVAPNNTSKTCSKCGHLNNYFNFEYRKKNKFPHFKCEKCNFKENADYNAALNISNPKLKSTKEEP

SEQ ID NO: 538 - protein, 726 aa, synthetic construct
GEDEFSHEYWMRHALTLAKRARDGREVPVGAVLVLNNRVIGEGWNRAIGLHDPTAHAEIMALRQGGLVMQNYRLIDATLYVTFEPCVMCAGAMVHSRIGRVVFGVRNSKRGAAGSLMNVLDYPGMGHRVEITEGILADECAALLCDFYRMPRQVFNARKKAQSSTNPGGSSGGSSGSETPGTSESATPGSSGGGSSGSAKNTITKTLQLRIVRPYNSAEVEKIVADEKNNREKIALEKNRDKVKEACSRHLEVAAYCTTQVERNACLFCKARKLDDKFYQGLRGQFPDAVFWQELGEIFRQLQRQAAEIYNQSLIELYYEIFIKGKGFANASSVEHYLSDVCYTRAAELFKNAAIASGLRGKVKSNFRLKELKSMKSGLPTTKSDNFPIPLVKQKGGQYTGFEISCHNDDFIIKIPFGRWQVKKEIDKYRPWEKFDFEQVRKSPKPISLLLSTQRRKKNKGWSKDEGTEAEIRRVMNGDYQTSYIEVKRGSRIGEKSAWMLSLSIDVPRIDKGVDPSIIGGIDVGVKSPLVCAINNAFGRYSISDNDLFHFNKKMFARRRILLKKNRHKRAGHGAKNKLKPITILTEKSKRFRKKLIERWACEIANFFIKNKVGTVQMENLEGMKRKEDSYFNIRLRGFWPYAEMQNKIEFKLKQYGIEIRKVAPNNTSKTCSKCGHLNNYFNFEYRKKNKFPHFKCEKCNFKENADYNAALNISNPKLKSTKGEP

SEQ ID NO: 539 - protein, 726 aa, synthetic construct
SEVEFSHEYWMRHALTLAKRARDEREVPVGAVLVLNNRVIGEGWNRAIGLHDPTAHAEIMALRQGGLVMQNYRLIDATLYVTFEPCVMCAGAMVHSRIGRVVFGVRNSKRGAAGSLMNVLNYPGMNHCVEITEGILADECAALLCDFYRMPRQVFNARKKAQSSINPGGSSGGSSGSETPGTSESATPESSGGSSGGSAKNTITKTLKLRIVRPYNSAEVEKIVADEKNSREKIALEKNKDKVKEACSEHLKVAAYCTTQVERNACLFCKARKLDDGFYQKLRGQFPDAVFWQEIGEIFRQLQKQAAEIYNQSLIELYYEIFIKGKGFANASSVEHYLSDVCYTRAAELFKNAAIASGLRGKVKSNFRLKELKNMKSGLPTTKSDNFPIPLVKQKGGQYTGFEISSHNDDFIIKIPFGRWQMKKEIDRYRPWEKFDFEQVRKSPKPISLLLSTQRRKRNKGWSKDEGTEAEIRKVMNGDYQTSYIEVKRGSKIGEKSAWMLSLSIDVPKIDKGVDPSIIGGIDVGVKSPLVCAINNAFSRYSISDNNLFHFNKKVFARRRILLKKNRHRRAGHGAKNKLKPITILTEKSKRFRKKLIERWACEIADFFIKNKVGTVQMENLESMKRREDSYFNIRLRGFWPYAEMQNKIEFKLKQYGIEIRKVAPNNTSRTCSKCGHLNNYFNFEYRKKNKFPHFKCEKCNFKEDADYNAALNISNPKLKSTKEES

SEQ ID NO: 540 - protein, 726 aa, synthetic construct
NEDEFSHEYWMRYALTLAKRARDGREVPVGAVLVLNNRVIGEGWNRAIGLHDPTAHAEIMALRQGGLVMQNYRLIDATLYVTFEPCVMCAGAMIHSRIGRVVFGVRNSKRGAAGSLMNVLNYPGMNHCVEITEGILVDECAALLCDFYRMPRQVLSAQKKAQSSVSSGGSSGGSSGSETPGTSESATPVSSSGSSGGSAKDTITKTLKLRVVRPYNSAEVEKIVADEKNNREKIALAKNKDKVKEACSEHLKVAAYCTTQVERNACLFCKARKLDDKFYQKLRGQFPDAVFWQEIGEVFRQLQKQAAEIYNQSLIELYYEIFIKGKGFANASSVEHYLSDVCYTRAAELFKNAAIASGLRGKVKSNFRLKELKNMKSGLPTTKSDNFPIPLVKQKGGQYTGFEISSHNDDFIIKIPFGRWQVKKEINKFRPWEKFDFEQVRKSPKPLSLLLSTQRRKRNKGWSKDEGTEAEIRKVMNGDYQISYIEVKRGSKIGEKNAWMLNLSIDVPKIDKGVDPSIIGGIDVGVKSPLVCAINNAFSRYSISDNDLFRFNKKLFARRRILLKKNRHKRAGHGAKNKLKPISILTEKSKRFRKKLIERWACEIADFFIKNKVGTVQMENLESMKRKEDSYFNIRLRGFWPYAEMQNKIEFKLKQYGIEIRKVAPNNTSKTCSKCGHLNNYFNFEYRKRNKFPHFKCEKCNFKENADYNAALNISNPKLKSTKEEP

SEQ ID NO: 541 - protein, 726 aa, synthetic construct
SEVEFSHEYWMRHALTLAKRARDEREVPVGAILVLNNRVIGEGWNRAIGLHDPTAHAEIMALRQGGLVMQNYRLIDATLYVTFEPCVMCAGAMIHSRIGRVVFGVRNSKHGAAGSLVNVLNYPGMNHRVEITEGILADECAALLCDFYRMPRRVFNAQKKAQSTINSGGSSGGSSGSETPGTSESPTPESSGGSPGGPAKNTITKTLKLRIVRPYNSTEVEKIVADEKNNREKIAIEKNKDMVKEACSKHLKVASYCTTQVERNACLFCKARKLDDKFYQKLRGQFPDAVFWQEIGEIFRQLQKQAAEIYNQSLIELYYEIFIKGKGFANASSVEHYLSDVCYTRAAELFKNAAIASGLRGKVKSNFRLKELKNMKSGLPTTKSDNFPIPLVKQKGGQYTGFEISSHNDDFIIKIPFGRWQVKKEIDKYRPWEKFDFEQVRKSPKPISLLLSTQRRKRNKGWSKDEGTEAEIRKVMNGDYQTSYIEVKRGSKIGEKSAWMLNLSIDVPKIDKGVDPSIIGGIDVGVKSPLVCAINNAFSRYSISDNDLFHFNKKMFARRRILLKKNRHKRAGHGAKNKLKPISILTEKSKRFRKKLIERWACEIANFFIKNKVGTVQMENLESMKRKGDSYFNIRLRGFWPYAEMQNKIEFKLKQYGIKIRKVAPNNTSKTCSKCGHLNNYFSFEYRKKNKFPHFKCEKCNFKEDADYNAALNISNPKLKSTKEEP

SEQ ID NO: 542 - protein, 726 aa, synthetic construct
SEVEFSHEYWMRHALALAKRARDAREVPVGAILVLNNRVIGEGWNRAIGQHDPTAHAEIMALRQGGLVMQNYRLIDATLYVTFEPCVMCAGAMIHSRIGRVVFGVRNSKHGAAGSLMNVLNYPGMNHRVEITEGILADECAALLCDFYRMPRQVFNGRKKAQSSINSGGSSGGSSGGETLGTREGATPESSGGSSGGSAKNTITKTLKLRIVRPYNSAEVEKIVVDEKNNREKVALEKNKDKVKEACSEHLKVAAYCTTQVERSACLFCKARKLDDKFYQKLRGQFPEAVFWQEIGEIFRQLQKQAAEIYNQSLIELYYEIFIKGKGFANASSVEHYLSDVCYTRAAELFKNAAIASGLRGKVKSNFRLKELKNMKSGLPTTKSDNFPIPLVKQKGGQYTGFEISSHNDDFIIKIPFGRWQVKKEIDKYRPWEKFDFEQVRKSPKPISLLLSTQRRKRNKGWSKDEGTEAEIKRVMNGDYQISYIEVKRGSKIGEKSAWMLSLSVDVPKIDKGVDPSIIGGIDVGVKSPLVCAINNALSRYSISDNDLFHFNKKMFARRRILLRNNRHKRAGHGAKSKLKPITILTEKGERFRKKLIERWACEIANFFIKNKVGTVQMENLESMKRKEDSYFNVRLRGFWPYAEMQNKIEFKLKQYGIEIRKVAPNNTSKTCSRCGHLNNYFNFEYRRKNKFPHFKCEKCNFEENADYNAALNISNPKLKSTKEEP

SEQ ID NO: 543 - protein, 726 aa, synthetic construct
SEVEFSHEYWMRHALTLAKRARDGREVPVGAVLVLNNRVIGEGWNRAIGLHDPTAHAEIMALRQGGLVMQNYRLIDATLYVTFEPCVMCAGAMVHSRIGRVVFGVRNSKRGAAGSLMNVLDYPGMGHRVEITEGILADECAALLCDFYCMPRRVFDAQKRAQSSINSGGSSGGSSGSETPGTSESATPESSGGGSSGSAKNTITKTLQLRIVRPYNSAEVEKIVADEKNNREKIALEKNKDKVKEACSKHLKVASYCTTQVERNACLFCKARKLDDKFYQKLRGQFPDAVFWQELGGIFRQLQKQAAEIYNQSLIELYYEIFIKGKGIANASSVEHYLSDVCYTRAAELFKNAAIASGLRNKIKSNFRLKELRNMKSGLPTTKSDNFPIPLVRQKGGQYTGFEISNHNGDFIIKIPFGRWQVKKEISKHRPWEKFDFEQVRKSPKPISLLLSTQRRKRNKGWGKDEGTEAEIRKVMNGDYQTSYIEVKRGSKIGEKSAWMLNLSIDVPKIDKGVDPSIIGGIDVGVKSPLVCAINNAFSRYSISDNDLFHFNKKMFARRRILLKKNRHKRAGHGVKNKLKPISILTEKSKRFRKKLIERWACEIADFFIKNKVGTVQMENLESMKRKEDSYFNIRLRGFWPYAEMQNKIEFKLKQYGIEIRKVAPNNTSKTCSKCGHLNNYFDFEYRKKNKFPRFKCEKCNFKENADYNAALNISNPKLKSTKEEP

SEQ ID NO: 544 - protein, 726 aa, synthetic construct
SEVEFSHEYWMRRALTLAKRARDEREVPVGAVLVLNNRVIGVGWNRAVGLHDPTAHAEIMALRQGGLVMQNNRLIEATLYVTFEPCIMCAGAMIHSRIGRVVFGVRNSKRGAAGSLMNVLNYPGMNHRVEITEGILADECAALLCDYYRMPRQVFNARKKAQSSINSGGSSDGGSSSETPGTSESATPESSGGSSGGSAKNTITKTLKLRIVRPYNSAEVEKIVADEKNNREKFALEKNKDKVKEACSEHLKVAAYCTTQVERSACLFCKARKLDDKFYQKLRGQFPDAVFWQEIGEIFRQLQKQAAEIYNQSLVELYYEIFIKGKGIANASSVEHYLSDVCYTRAAELFKNAAIASGLRNKIKSNFRLKELRNMKSGLPTTKSDNFPIPLVRQKGGQYTGFEISDHDGDFIIKIPFGRWQVKKEINKHRPWEKFDFEQVRKSPKPISLLLSTQRRKRNKGWSKDEGTEAEIRKVMNGDYQTSYIEVKRGSKIGEKSAWMLNLSIDVPKIDKGVDPSIIGGIDVGVKSPLVCAINNALSRYSISDNDLFHFNKKMFARRRILLRKNRHKRAGHGAKNKLKPITMMTEKSKRFRKKLIERWACEIADFFVKNKVGTVQMENLESMKRKEDSYFNIRLRGLWPYAEMQNKIEFKLKQYGIEIRKVAPNNTSKTCSKCGHLNNYFNFEYRKKNKFPHFKCEKCNFKENADYNAALNISNPKLKSTKEEP

SEQ ID NO: 545 - protein, 726 aa, synthetic construct
SEVEFSHEYWMRRALTLAKRARDEREVPVGAVLVLNNRVIGVGWNRAVGLHDPTAHAEIMALRQGGLVMQNYRLTEATLYVTFEPCIMCAGAMIHSRIGRVVFGVRNSKRGAAGSLMNVLNYPGMNHRVEITEGILADECAALLCDFYCMPRQVLNAQKKARSCINSGGSSGGSSGSETPGTSESATPESSGGSSGGSAKNTITKTLKLRIVRPYNSAEVEKIVADEKNNREKIALEKNKDKVKEACSKHLKVASYCTTQVERNACPFCKARKLDDKFYQKLRGQFPDAVFWQELGGIFRQLQKQAAEIYNQSLIELYYEIFIKGKGITNASRVEHYLSDVCYTRAAELFKNAAIASGLRSKVRSNFRLKELKNMKSGLPTTKSDNFPIPLVKQKGGQYTGFEISSHNSDFIIKIPFGRWQEKEEIDKYRPWEKFDFEQVRRSPKPISLLLSTQRRKKNKGWSKDEGTEAEIRKVMNGDYQTSYIEVKRGSKTGEKSAWMLNLSIDVPKIDKGVDPSTIGGIDVGVKSPLVCAINNAFSRYSISDNDLFRFNKKMFARRRILLKKNRHKRAGHGAKNKLKPITILTEKSRRFRKKLIERWACEIADFFIKNKVGTVQMESLESMKRKEDSYFNTRLRGFWPYAEMQNKIEFKLKQYGIKVRKVAPNNTSKTCSKCGHLNNYFSFEYRKKNKFPHFKCEKCNFKENADYNAALNISNPKLKSTKEEP

SEQ ID NO: 546 - protein, 726 aa, synthetic construct
SEVEFSHEYWMRHALTLAKRARDEREVPVGAVLVLNNRVIGEGWNRAIGLHDPTAHAEIMALRQGGLVMQNHRLVDATLYVTFEPCVMCAGAMIHSRIGRVVFGVRNSKRGAAGSLMNVLNYPGMNHYVEITEGILVDECAALLCDFYRMPRQVLNAQKKAQSSINPGGSSGGSSGSETPGTSESATPESSGGSSGSSAKNTITKTLKLRIVRPYNSAEVEKIVADEKNNREKIALEKNKDKVKEACSKHLKVAAYCTTQVERNACLFCKARRLDDKFYQKLRGQFPDAVFWQEIGEIFRQLQKQAAEVYNQSLVELYYEILIKGKGIANASSVEHYLSDVCYTRAAELFKNAAIASGLRNKIKSNFRLKELRNMKSGLPTTKSDNFPIPLVRQKGGQYTGFEISNHDGDFIIKIPFGRWQAKKEINKHRPWEKFDFEQVRKSPKPISLLLSTQRRKRNKGWSKDEGTEAEIRKVMNGDYQTSYIEVKRGSKIGEKSAWMLNLSIDVPKIDKGVDPSIIGGIDVGVKSPLVCAINNALSRYSISDNDLFHFNKKMFARRRILLRKNRHKRAGHGAKNKLKPITIMTEKSKRFRKKLIERWACEIADFFIKNKVGTVQMENLESMKRKEDSYFNIRLRGFWPYAEMQNKIEFKLKQYGIVVRKVAPNNTSKTCSKCGHLNNYFNFEYRKKNKFPHFKCEKCNFKEDADYNAALNISNPKLKSTKEEP

SEQ ID NO: 547 - protein, 726 aa, synthetic construct
GEDEFSHEYWMRHALTLAKRARDGREVPVGAVLVLNNRVIGEGWNRAIGLHDPTAHAEIMALRQGGLVMQNYRLIDATLYVTFEPCVMCAGAMIHSRIGRVVFGVRNSKHGAAGSLVNVLNHPGMNHRVEITEGILADECAALLCDFYRMPRQVFNARKKAQSSINPGGSSGGSSGSETPGTSESATPESSGGSSGGSAKNTITKTLKLRIVRPYNSAEVEKIVADEKNSREKIALERNKDKVKEACSEHLKVASYCTTQVERNACPFCKARKLDDKFYQKLRGQFPDAVFWQELGEILRQLQKQAAEIYNQSLIELYYEIFIKGRGFANASSVEHYLSDVCYTRAAELFKNAAIASGLRGKVKGNFRLKELKNMKSGLPTTKSDNFPIPLVKQKGGQYTGFEISNHNGDFIIKIPFGRWQVKKEINKYRPWEKFDFEQVRKSPKPISLLLSTQRRKRNKGWSKDEGTEAEIRKVMNGDYQTSYIEVKRGSKIGEKSAWMLNLSIDVPKIDKGVDPSIIGGIDVGVKSPLVCAINNALSRYSISDNDLFHFNKKMFARRRILLRKNRHKRAGHGAKNKLKPITMMTEKSKRFRKKLIERWACEIADFFIKNKVGTVQMENLESMKRKEDSYFNIRLRGFWPYAEMQNKIEFKLKQYGIEVRKVAPNNTSKTCSKCGHLNNYFGFEYRKKNKFPHFKCEKCNFKEDADYNAALNISNPKLKSTKEEP

SEQ ID NO: 548 - protein, 726 aa, synthetic construct
SEVEFSHEYWMRHALTLAKRARDEREVPVGAILVLNNRVIGEGWNRAIGLHDPTAHAEIMALRQGGLVMQNYRLIDATLYVTFEPCVMCAGAMIHSRIGRVVFGVRNNKHGAAGSLVNVLNYPGMNHRVEITEGILADECAALLCDFYRMPRQVFNARKKAQSSINPGGSSGGSSGSETPGTSESATPESSGGSSGSSAKNTITKTLKLRIVRPYNSAEVEKIVADEKNNREKIALEKNKDKVKEACSKHLKVAAYCTTQVERSACLFCKARKLDDKFYQKLRGQFPDAVFWQEIGEIFRQLQKQAAEIYNQSLIELYYEIFIKGKGFANASSVEHYLSDVCYTRAAELFKNAAIASGLRGKVKSNFRLKELKNMKSGLPTTKSDNFPIPLVKQKGGQYTGFEISSHNDDFIIKIPFGRWQVKKEIDKYRPWEKFDFEQVRKSPKPISLLLSTQRRKRNKGWSKDEGTEAEIRKVMNGDYQTSYIEVKRGSKIGEKSAWMLNLSIDVPKIDKGVDPSIIGGIDVGVKSPLVCAINNAFSRYSISDNDLFRFNKKVFARRRILLKKNRHKRAGHGTKNKLKPITILTEKSGRFRKKLIERWACEIANFFIKNKVGTVQMENLESMKRKEDSYFNIRLRGFWPYAEMQNKIEFKLKQYGIKIRKVAPNNTSKTCSKCGHLNNYFNFEFRKKNKFPHFKCEKCNFKENADYNAALNISNPKLKSTKEEP

SEQ ID NO: 549 - protein, 726 aa, synthetic construct
SEVEFSHEYWMRHALTLAKRARDEREVPVGAVLVLNNRVIGEGWNRAIGLHDPTAHAEIMALRQGGLVMQNYRLSDATLYVTFEPCVMCAGAMIHSRIGRVVFGVRNSKRGAAGSLMNVLNYPGMNHCVEITEGILVDECAALLCDFYRMPRQVLSAQKKAQSSISSGGSSGGSSGSETPGARGSVTPKSSGGGSSGSAKNTITKTLQLRIVRPYNSAEVEKIVADEKNNREKIALEKNKDKVKEACSKHLKVASYCTTQVERNACLFCKARKLDDKFYQKLRGQFPDAVFWQELGEILRQLQKQAAEIYNQSLIELYYEIFIKGRGFANASSVEHYLSDVCYTRAAGLFKNAAIASGLRGKVKSNFRLKELKNMKSGLPTTKSDNFPIPLVRQKGGQYTGFEISNHDGDFIIKIPFGRWQVKKEADKYRPWEKFDFEQVRKSPKPISLLLSTQRRKRNKGWSKDGGTEAEIKKVMSGDYQTSYIEVKRGSKIGEKSAWMLSLSIDVPKIDRGVDPSIIGGIDVGVRSPLVCAINNASSRLSISDNDLFRFNKKMFARRRILLKKNGHKRAGHGAKNKLKPITVLTEKSERFRKKLIERWACEIANFFIKNKVGTVQMENLESMKRREDSYFNIRLRGFWPYAEMQNKIEFKLKQYGVAIRKVAPNNTSKTCSKCGHLNNYFNFEYRKKNKFPHFKCEKCNFKENADYNAALNISNPKLKSTKEEP

SEQ ID NO: 550 - protein, 726 aa, synthetic construct
SEVEFSHEYWMRRALTLAKRARDEREVPVGAVLVLNNRVIGEGWNRAIGLHDPTAHAEIMALRQGGLVLQNYRLVDATLYVTFEPCVMCAGAMVHSRIGRVVFGVRNSKRGAAGSLMNVLDHPGMDHRVEITEGILADECAALLCDFYRMPRQVFNARKKAQSSINSGGSSDGGSGSETPGTSESATPESSGGSSGGSAKNTITKALKLRIVRPFNSAEVEKIVADEKNNREKIALEKNKDKVKEACSEHLKVAAYCTTQVERSACLFCKARKLDDKFYQKLRGQFPDAVFWQEIGEIFRQLQKQAAEIYNQSLIELYYEIFIKGKGFANACSVEHYLSDVCYTRAAELFKNAAIASGLRGKVKSNFRLKELKNMKSGLPTTKSDNFPIPLVKQKGGQYTGFEISSHNDDFIIKIPFGRWQVKKEIDKYRPWEKFDFEQVRKSPKPISLLLSTQRRKRNKGWSKDEGTEAEIRKVMNGDYQTSYIEVKRGSKIGEKSAWMLNLSIDVPKIDKGVDPSIIGGIDVGVRSPLVCAINNAFSRYSISDNDLFRFNKKMFARRRILLKKNRHKRAGHGAKNKLKPITILTEKSRRFRKKLIERWACEIADFFIKNKVGTVQMESLEGMKRKEDSYFNVRLRGFWPYAEMQNKIEFKLKQYGIKIRKVAPNNTSKTCSMCGHLNNYFSFEYRKKNKFPHFKCEKCNFKENADYNAALNISNPKLMSTKEGP

SEQ ID NO: 551 - protein, 726 aa, synthetic construct
SEVEFSHEYWMRHALTLAKRARDEREVPVGAVLVLNNRVVGEGWNRAIGLHDPTAHAEIMALRQGGLVMQNYRLTDATLYVTFEPCVMCAGAMIHSRIGRVVFGVRNSKRGAAGSLMNVLNYPGMNHCVEITEGILVDECAALLCDFYRMPRQVLSAQKKAQSSISSGGSSGGSSGSETPGASGSVTPKSSVGSSAGSTKNTITKTLKLRIVRPYNSAEVEKIVADEKNNREKIALEKNKDKVKEACGKHLKMASYCTTQVERNACLFCKARKLDDKFYQKLRGQFPDAVFWQELGGIFRQLQKQAAEIYNQSLIELYYEIFIKGKGITNASRVEHYLSDVCYTRAAELFKNAAIASGLRSKVRSNFRLKELKNMKSGLPTTKSDNFPIPLVKQKGGQYTGFEISNHNSDFIIKIPFGRWQVKEEINKYRPWEKFDFEQVRKSPKPISLLLSTQRRKRNKGWSKDEGTEAEIRKVMNGDYQTSYIEVKRGSKVGEKSAWMLNLSIDVPKIDKGVNPSIIGGIDVGVKSPLVCAINNALSRYSISDNDLFHFNKKMFARRRILLKKNRHKRAGHGAKNKLKPITILTGKCKRFRKKLIERWACEIADFFIKNKVGTVQMENLESMKRKEDSYFNIRLRGFWPYAEMQNKIEFKLKQYGIEIRKVAPNNTSKTCSKCGHLNNYFNFEYRKRNKFPHFKCEKCNFKENADYNAALNISNPKLKSTKEEP

SEQ ID NO: 552 - protein, 726 aa, synthetic construct
SEVEFSHEYWMRRALTLAKRARDEREVPVGAVLVLNNRVIGVGWNRAVGLHDPTAHAEIMALRQGGLVMQNYRLIEATLYVTFEPCIMCAGAMIHSRIGRVVFGVRNSKRGAAGSLMNVLNYPGMNHRVEITEGILADECAALLCDYYRMPRQVFNARKKAQSSISSGGSSEGSGGGETPGASESVTPKSSGGSSAGSTKNTITKTLKLRIVRPYNSAEVEKIVADEKNSREKIALEKNKDKVKEACSEHLKVAAYCTTQVERSACLFCKARKLDDRFYQKLRGQFPDAVFWQEISEIFRQLQKQAAEIYNQSLIELYYEILIKGKGIANAGRVEHYLSDVCYTRAAELFKNAAIASGLRSKIKSNFRLKELRNMKSGLPTTKSDNFPIPLVKQKGGQCTGFEINSHNDDFIIKIPFGRWQVKEEIDKYRPWEKFDFEQVRKSPKPISLLLSTQRRKKNKGWSKDEGTEAEIRRVMNGDYQTSYIEVKRGSKIGEKSAWMLNLSIDVPKVDKGVDPSIIGGIDVGVKSPLVCAINNSSSRYSICDNDLFRFNKKMFARRRILLKKNRHKRAGHGAKNKLKPITILTEKSVRFRKKLIERWACEIADFFVKNKVGTVQMENLESMKGKEDSYFNIRLRGFWPYAEMQNKIEFKLKQYGIEIRKVAPNNTSKTCSKCGHLNNYFNFEYRKKNKFPHFKCEKCYFKEDADYNAALNISNPKLKNTKGEP

SEQ ID NO: 553 - protein, 726 aa, synthetic construct
SEVEFSHEYWMRHALSLAKRARDEREVPVGAVLVLNNRIIGEGWNRAIGLHDPTAHAEIMALRQGGLVMQNYRLTDATLYVTFEPCVMCAGAMVHSRIGRVVFGVRNSKRGAAGSLMNVLNYPGVNHCVEITEGILVDECAALLCDFYRMPRQVLNAQKKAQSSISSGGPSGGCSGSEMPGASGSVTPKSSGGSSAGSTKNTITKTLKLRIVRPYNSAEVEKIVADEKNNREKVALEKNKDKVKEACSKHLKMAAYCTTQVERNACLFCKARRLDDKFYQKLRGQFSDAVFWQEIGEIFRQLQKQAAEIYNQSLIELYYEIFIKGKGFANASSVEHYLSDVCYTRAAELFKNAAIASGLRGKVKSNFRLKELKNMKSGLPTTKSDNFPIPLVKQKGGQYTGFEISSHNDDFIIKIPFGRWQAKKEIDKYRPWEKFDFEQVRKSPKPISLLLSTQRRKRNKGWSKDEGTEAEIRKVMNGDYQTSYIEVKRGSKIGEKSAWMLYLSIDVPKIDKGVDPSIIGGIDVGVKSPLVCAINNAFSRYSISDNDLFRFNKKMFARRRILLKKNRHKRAGHGAKNKLKPITVLTEKSGRFRKKLIERWACEVANFFIKNKVGTVQMESLESMKRREDSYFNIRLRGFWPYAEMQNKIEFKLKQYGIEVRKVAPNNTSKTCSKCGHLNNYFNFEYRKKNKFPLFKCEKCNFKENADYNAALNISNPKLKSTREEP

SEQ ID NO: 554 - protein, 726 aa, synthetic construct
SEVEFSHEYWMRHALTLAKRARDEREVPVGAILVLNNRVIGEGWNRAIGLHDPTAHAEIMALRQGGLVMQNYRLTDATLYVTFEPCVMCAGAMIHSRIGRVVFGVRNSKRGAAGSLMNVLNYPGMNHCVEITEGILVDECAALLCDFYRMPRQVLSAQKKAQSSIGPGGSSGGSSGSETPGASGSVTPKSSGGSSAGSTKDTITKTLKLRIVRPYNSAEVEKIVADEKNSREKIALEKNKDKVKEACSEHLKVAAYCTTQVERNACLFCKARKLDDKFYQKLRGQFPDAVFWQELGEIFRQLQKQAAEIYNQSLIELYYEIFIKGKGFANASSVEHYLSDVCYTRAAELFKNAAIASGLRGKVKSNFRLKELRNMKSGLPTTKSDNFPIPLVRQKGGQYTGFEISSRNDDFIIKIPFGRWQVKKEIDKYRPWEKFDFEQVRKSPKPISLLLSTQRRKRNKGWSKDEGTEAEIRKVMNGDYQTSYIEVKRGSKIGEKSAWMLNLSIDVPKIDKGVDPSIIGGIDVGVKSPLVCAINNALSRYSISDNDLFHFNKKMFARRRILLRKNRHKRAGHGARNKLKPITVLTEKSERFRKKLIERWACEIANFFIKNKVGTVQMENLESMKRREDSYFNIRLRGFWPYAEMQSKIEFKLKQYGIKIRKVAPNNTSKTCSKCGHLNNYFNFEFRKKNKFPHFKCEKCNFKEDADYNAALNISNPKLKSTKEEP

SEQ ID NO: 555 - protein, 726 aa, synthetic construct
SEVEFSHEYWMRHALALAKRARDEREVPVGAVLVLNNRVIGEGWNRAIGLHDPTAHAEIMALRQGGLAMQNYRLVDATLYVTFEPCVLCAGAMVHSRIGRVVFGVRNSKRGAAGSLMNVLNHPGMNHRVEITEGILVDECAALLCDFYRMPRQVLNAQKKAQSSISSGGSSGGSSGSETPGASESVTPKSSGGSPGGSAKNTITKTLKLRIVRPYNSAEVEKIVADEKNNREKIALEKNKDKVKEACSKHLKMASYCTTQVERNACLFCKARKLDDKFYRKLRGQFPDAVFWQELGGILRQLQKQAAEIYNQSLIELYYEIFIKGKGITNASRVEHYLSDVCYTRAAELFKNAAIASGLRSKVRSNFRLKELKNMKSGLPTTKSDNFPIPLVKQKGGQYTGFEISSHNSDFIIKIPFGRWQVKEEIDKYRPWEKFDFEQVRKSPKPISLLLSTQRRKRNKGWSKDEGTEAEIRRVMNGDYRTSYIEVKRGSKIGEKSAWMLNLSIDVPKIDKGVDPSIIGGIDVGVKSPLVCAINNSSSRYSICDNDLFRFNKKMFARRRILLKKNRHKRAGHGAKNKLKPITILTKKSERFRKKLIERWVCEVADFFIKNKVGTVQMENLESMKRKEDSYFNIRLRGFWPYAEMQNKIEFKLKQYGIVVRKVAPNNTSKTCSKCGHLNNYFNFEYRKKNKFPHFKCEKCNFKEDADYNAALNISNPKLKSTKGEP

SEQ ID NO: 556 - protein, 726 aa, synthetic construct
SEVEFSHEYWMRHALTLAKRARDEREVPVGAVLVLNNRVIGEGWNRAIGMHDPTAHAEIMALRQGGLVMQNYRLVDATLYVTFEPCVLCAGAMVHSRIGRVVFGVRNSKRGAAGSLMNVLNYPGMNHRVEITEGILADECAALLCDFYRMPRRVFNARKKAQSSTNPGGSSGGSSGSETPGTSESATPESSGGGSSGSAKNTITKTLQLRIVRPYNSAEVEKVVADEKNNREKIALEKNKDKVKEACSKHLKVASYCTTQVERNACPFCKARKLDDKFYQKLRGQFPDAVFWQELGEILRQLQKQAAEIYNQSLIELYYEIFIKGRGFANASSVEHYLSDVCYTRAAELFKNAAIASGLRGKVKSNFRLKELKNMKSGLPTTKSDNFPIPLVKQKGGQYTGFEISSHNDDFIIKIPFGRWQVKKEIDRYRPWEKFDFEQVRKSPKPISLLLSTQRRKRNKGWSKDEGTEAEIRKVMNGDYQTSYIEVKRGSKIGEKSAWMLNLSIDVPKIDKGVDPSIIGGIDVGVKSPLVCAINNAFSRYSISDNDLFRFNKKMFARRRILLKKNRHKRAGHGAKNKLKPITILTEKSVRFRKKLIERWACEIADFFIKNKVGTVQMENLESMKRKEDSYFNIRLRGFWPYAEMQNKIEFKLKQYGIEIRKVAPNNTSKTCSKCGHLNNYFNFEYRKKNKFPHFKCEKCNFKENADYNAALNISNPKLKSTKEEP

SEQ ID NO: 557 - protein, 726 aa, synthetic construct
SEVEFSHEYWMRHALTLAKRARDEREVPVGAILVLNNRVIGEGWNRAIGLHDPTAHAEIMALRQGGLVMQNYRLIDATLYVTFEPCVMCAGAMIHSRIGRVVFGVRNSKHGAAGSLVNVLNYPGMNHRVEITEGILADECAALLCDFYRMPRQVFNARKKAQSSINPSGSSGGSSGSVTPGTSESATPESSGGGFGGSAKNTITKTLQLRIVRPYNSAEVEKIVADEKNNREKIALEKNKDKVKEACSKHLKVASYCTTQVERNACLFCKARKLDDKFYQKLRGQFPDAVFWQETGEIFRQLQRQAAEIYNQSLIELYYEIFIKGKGFANASSVEHYLSDVCYTRAAELFKNAAIASGLRGKVKGNFRLKELKNMKSGLPTTKSDNFPIPLVKQKGGQYTGFEISSHNSDFIIKIPFGRWQVKKEIDKYRPWEKFDFEQVRKSPKPISLLLSTQRRKRNKGWSKDEGTEAEIRKVMNGDYQTSYIEVKRGSKTGEKSAWMLNLSIDVPKIDKGVDPSIIGGIDVGVKSPLVCAINNAFSRYSISDNDLFRFNKKMFARRRILLKKNRHKRAGHGAKNKLKPITIMTEKSKRFRKKLIERWACEIADFFIKNKVGTVQMENLESMKRKEDSYFNIRLRGFWPYAEMQDKIEFKLKQYGIEIRKVAPNNTSKTCSRCGHLNNYFNFEYRKKNKFPHFKCEKCNFKEDADYNAALNISNPKLKSTKGEP

SEQ ID NO: 558 - protein, 726 aa, synthetic construct
SEVEFSHEYWMRHALTLAKRARDEHEVPVGAILVLNNRVIGVGWNRAIGLHDPTAHAEIMALRQGGLVTQNYRLIDATLYVTFEPCVMCAGAMIHSRIGRVVFGVRNSKHGAAGSLVNVLNYPGMNHRVEITEGILADECAALLCDFYRMPRQVFNARKKAQSSINSGGSSGGSSGSETPGTSESVTPKSSVGSSASSTKNTITKTLKLRIVRPYNSAEVEKIVADEKDNREKIALEKNKDKVKEACSKHLKVAAYCTTQVERNACLFCKARKLDDRFYQKLRGQFPDAVFWQETGEIFRQLQRQAAEIYNQSLIELYYEIFIKGKGFANASSVEHYLSDVCYTRAAELFKNAAIASGLRGKVKSNFRLKELKNMKSGLPTTKSDNFPIPLVKQKGGQYAGFEISSHNDDFIIKIPFGRWQVKKEIDKYRPWEKFDFEQVRKSPKPISLLLSTQRRKRNKGWSKDEGTEAEIRKVMNGDYQTSYIEVKRGSKIGEKSAWMLSLSIDVPKIDKGVDPSIIGGIDVGVKSPLVCAINDAFSRYSISDNDLFHFNKKMFARRRILLKKNGHKRAGHGAKNKLKPITIMTEKGKRFRKKLIERWACEIADFFIKNKVGTVQMENLESMKRKEDSYFNIRLRGFWPYAEMQNKIEFKLKQYGIKVRKVAPNNTSKTCSKCGHLNNYFSFEYRKKNKFPHFKCEKCNFKENADYNAALNISNPKLKSTKEEP

SEQ ID NO: 559 - protein, 726 aa, synthetic construct
SEVEFSHEYWMRHALSLAKRARDEREVPVGAVLVLNNRIIGEGWNRAIGLHDPTAHAEIMALRQGGLVMQNYRLTDATLYVTFEPCVMCAGAMVHGRIGRVVFGVRNSKRGAAGSLMNVLNYPGVNHCVEITEGILVDECAALLCDFYRMPRQVLNAQKKAQSSISSGGSSGGCSGSEMPGASESVTPKSSGGSSAGSTKNTITKTLKLRIVRPYNSAEVEKIVADEKNSREKIALERNKDKVKEACSEHLKVAAYCTTQVERNACLFCKARKLDDRFYQKLRGQFPDAVFWQEIGEIFRQLQKQAAEIYNQSLIELYYEIFIKGRGFANASSVEHYLSDVCYTRAAELFKNAAIASGLRGKVKSNFRLKELKNMKSGLPTTKSDNFPIPLVKQKGGQYTGFEISSHNDDFIIKIPFGRWQVKKEIDKYRPWEKFDFEQVRKSPKPISLLLSTQRRKRNKGWSKDEGTEAEIRRVMSGDYQTSYIEVKRGSKIGEKSAWMLNLSIDVPKIDKGVDPSIIGGIDVGVKSPLVCAINDAFSRYSISDNDLFRFNKKMFARRRILLGKNRHKRAGHGVKNKLKPITILTEKSKRFRKKLIERWACEIADFFIKNKVGTVQMENLESMKRKEDSYFNIRLRGFWPYAEMQNKIEFKLKQYGIEIRKVAPNNTSKTCSKCGHLNNYFNFEYRRKNKFPHFKCEKCNFKENADYNAALNISNPKLKSTKGEP

SEQ ID NO: 560 - protein, 726 aa, synthetic construct
SEVEFSHEYWMRHALTLAKRARDEREVPVGAILVLNNRVIGVGWNRAIGLHDPTAHAEIMALRQGGLVMQNYRLIDATLYVTFEPCVMCAGAMIHSRIGRVVFGVRNSKHGAAGSLVNVLNYPGMNHRVEITEGILADECAALLCDFYRMPRQVFNARKKAQSSINSGGSSGGSSGSETPGTSESATPKSSGGSSGGSAKNTITKTLKLRIVRPYNSAEVEKIVADEKNSREKIALEKNKDKVKEACSEHLKVAAYCTTQVERNACLFCKARKLDDKFYQKLRGQFPDAVFWQEIGEIFRQLQKQAAEVYNQSLVELYYEILIKGKGIANASSVEHYLSDVCYTRAAELFKNAAIASGLRNKIKSNFRLKELRNMKSGLPTTKSDNFPIPLVRQKGGQYTGFEISNHDGDFIIKIPFGRWQVKKEINKHRPWEKFDFEQVRKSPKPISLLLSTQRRKRNKGWSKDEGTEAEVRKVMNGDYQTSYIEVKRGSKIGEKSAWMLNLSIDVPKIDKGVDPSIIGGIDVGVKSPLVCAINNALSRYSISDNDLFHFNKKMFARRRILLRKNRHKRAGHGAKNKLKPITIMTEKSKRFRKKLIERWACEIADFFIKNKVGTVQMENLESMKRKEDSYFNIRLRGFWPYAEMQNKIEFKLKQYGIEIRKVAPNNTSKTCSKCGHLNNYFNFEYRKMNKFPHFKCEKCNFKENADYNAALNISNPKLKSTKEEP

SEQ ID NO: 561 - protein, 726 aa, synthetic construct
SEVEFSHEYWMRHALTLAKRARDEREVPVGAILVLNNRVIGEGWNRAIGLHDPTAHAEIMALRQGGLVMQNYRLIDATLYVTFEPCVMCAGAMIHSRIGRVVFGVRNSKHGAAGSLVNVLNYPGMNHRVEITEGILADECAALLCDFYRMPRQVFNARKKAQSSISPGGSSGGSSGSETPGTSESATPESSGGSPGGSAKNTITKTLKLRIVRPYNSAEVEKIVADEKNNREKIALEKNKDKVKEACSKHLKVAAYCTTQVERNACLFCKARKLDDKFYQKLRGQFPDAVFWQEIGEIFRQLQKQAAEIYNQSLIELYYEIFIKGKGFANASSVEHYLSDVCYTRAAELFKNAAIASGLRGKVKSNFRLKELKNMKSGLPTTKSDNFPIPLVKQKGGQYTGFEISSHNDDFIIKVPFGRWQAKKEIDKYRPWEKFDFEQVRKSPKPISLLLSTQRRKRNKGWSKDEGTEAEIKKVMSGDYQTSYIEVKRGSKTGEKSAWMLNLSIDVPKIDKGVDPCIIGGIDVGVKSPLVCAINNAFSRYSISDNDLFRFNKKVFARRRILLKKNRHKRAGHGTKNKLKPITILTEKSGRFRKKLIERWACEIANFFIKNKVGTVQMENLESMKRKEDSYFNIRLRGFWPYAEMQNRIEFKLKQYGIKIRRVAPNNTSKTCSKCGHLNNYFSFEYRKKNKFPHFKCEKCNFKEDADYNAALNISNPKLKSTKEEP

SEQ ID NO: 562 - protein, 726 aa, synthetic construct
SEVEFSHEYWMRHALTLAKRARDEREVPVGAILVLNNRVIGEGWNRAIGLHDPTAHAEIMALRQGGLVMRNYRLTDATLYVTFEPCVMCAGAMIHSRIGRVVFGVRNSKRGAAGSLMNVLNYPGMNHCVEITEGILVNECAALLCDFYRMPRQVLNAQKKAQSSISPGGSSGGSGGSETPGASESVTPKSSGGSSGGSAKNTITKTLKLRIVRPYNSAEVEKIVADEKNNREKIALEKNKGKVKEACSKHLEVAAYCTTQVERNACLFCKARKLDDKFYQKLRGQFPDAVFWQELGEIFRQLQKQAAEIYNQSLIELYYEIFIKGKGFANASSVEHYLSDVCYTRAAELFKNAAIASGLRGKVKSNFRLKELKNMKSGLPTTKSDNFPIPLVKQKGGQYTGFEISSHNDDFIIKIPFGRWQVKKEIDKYRPWEKFDFEQVRKSPKPISLLLSTRRRKRNKGWSKDEGTEAEIRRVMNGDYQTSYIEVKRGSKIGEKSAWMLNLSIDVPKIDKGVDPSIIGGIDVGVKSPLVCAINNSSSRYSISDNDLFHFNKKVFARRRILLKKNRHRRAGHGAKNKLKPITILTEKSKRFRKKLIERWACEIADFFIKNKVGTVQMENLESMKRKEDSYFNIRLRGFWPYAEMQNKIEFKLKQYGIKVRKVAPNNTSRTCSECGHLNNYFSFEYRKKNKFPHFKCKKCNFKEDADYNAALNISNPKLKGTKEEL

SEQ ID NO: 563 - protein, 726 aa, synthetic construct
SEVEFSHEYWMRHALTLAKRARDEREVPVGAVLVLNNRVIGEGWNRAIGLHDPTAHAEIMALRQGGLVMQNYRLTDATLYVTFEPCIMCAGAMIHSRIGRVVFGVRNSKRGAAGSLMNVLNYPGMNHCVEITEGILVDECAALLCDFYRMPRQVLNAQKKAQSSISSGGSSGGSSGRETPGASGSVTPKSSGGSSGGSAKNSITKALKLRIVRPYNSAEVEKIVADEKNNREKTALEKNKGKVKEACSKHLKVATYCTTQVERNACLFCKARKLDDKFYQKLRGQFPDAVFWQEIGEIFRQLQKQAAEIYNQSLIELYYEIFIEGKGSANARSVEHYLSDVCYTRAAELFKNAAIASGLRGKVKGNFRLKELKSMKSGLPTTKSDNFPIPLVKQKGGQYTGFEISSHNDDFIIKIPFGRWQVKKEIDKYRPWEKFDFEQVRKSPKPISLLLSTQRRKRNKGWSKDEGTEAEIRKVMNGDYQTSYIEVKRGSKIGEKSAWMLNLSIDVPKIDKGVDPGIIGGIDVGVKSPLVCAINNAFSRYSISDNDLFHFNKKMFARRRILLKKNRHKRAGHGAKNKLKPISILTEKSKRFRKKLIERWACEIADFFIKNKVGTVQMENLESMKRKEDSYFNIRLRGFWPYAEMQNKIEFKLKQYGIEIRKVAPNNTSKTCSKCGHLNNYFNFEYRKKNKFPHFKCEKCNFKENADYNAALNISNPKLKSTKEEP

SEQ ID NO: 564 - protein, 726 aa, synthetic construct
SEVEFSHEYWMRHALTLAKRARDEREVPVGAVLVLNNRVIGEGWNRAIGLHDPTAHAEIMALRQGGLAMQNYRLVDATLYVTFEPCVLCAGAMVHSRIGRVVFGVRNSKRGAAGSLMNVLNHPGMNHRVEITGGILADECAALLCDFYRMPRQVFNAQKKARSNINSGGSSGGSSGSETLGTSESATPESSGGSSGGSAKNTITKALKLRIVRPYNSAEVEKIVADEKNNREKIALEKNKDKVKEACSKHLKVASYCTTQVERNACPFCRARKLDDKFYQKLRGQFPDAVFWQELGEILRQLQKQAAEIYNQSLIELYYEIFIKGKGFANASSVEHYLSDVCYTRAAELFKNAAIASGLRGKVKSNFRLKELKNMKSGLPTTKSDNFPIPLVKQKGGQYTGFEISNHNSDFIIKIPFGRWQVKKEINKYRPWEKFDFEQVRRSPKPISLLLSTQRRKRNKGWSKDEGTEAEIRKVMNGDYQTSYIEVKRGSRIGEKSAWMLSLSIDVPKIDRGVDPSIIGGIDVGVKSPLVCAINNALSRYSISDNDLFHFNKKMFARRRILLKKNRHRRAGHGARNKLKPITVLTEKSKRFRKKLIERWACEIASFFIKNKVGTVQMENLESMKRKEDSYFNIRLRGLWPYAEMQNKIEFKLKQYGIEIRKVAPNNTSKTCSKCGHLNNYFNFEYRKRNKFPHFKCEKCNFKENADYNAALNISNPNLKGTKEEP

SEQ ID NO: 565 - protein, 726 aa, synthetic construct
SEVEFSHEYWMRHALTLAKRARDEREVPVGAVLVLNNRVIGEGWNRTTGLHDPTAHAEIMALRQGGLVMRNYRLTDATLYVTFEPCVMCAGAMIHSRIGRVVFGVRNSKRGAAGSLMNVLNYPGMNHRVEITEGILVDECAALLCDFYRMPRQVLNAQKKAQSSISSGGSSGGSSGNETPGASESATPKSSSGSSAGSTKNTITKTLKLRIVRPYNSAEVEKIVADEKNNREKIALEKNKDKVKEACSKHLKVASYCTTQVERNACPFCKARKLDDKFYQKLRGQFPDAVFWQELGEILRQLQKQAAEIYNQSLIELYYEIFIKGRGFANASSVEHYLSDVCYTRAAELFKNAAIASGLRGKVKSNFRLKELKNMKSGLPTTKSDNFPIPLVKQKGGQYTGFEISSHNNDFIIKIPFGRWQVKEEIDKYRPWEKFDFEQVRKSPKPISLLLSTQRRKKNKGWSKDEGTEAEIRKVMNGDYQTSYIEVKRGSKTGEKSAWMLNLSIDVPKIDKGVDPSIIGGIDVGVKSPLVCAINNAFSRYSISDNDLFRFNKKMFARRRILLKKNRHKRAGHGAKNKLKPISILTGKSERFRKKLIERWACEIADFFIKNKVGTVQMENLESMKRKEDSYFNIRLRGFWPYAEMQNKIEFKLKQYGIKIRKVAPNNTSKTCSKCGHLNNYFNFEYRKKNKFPHFKCEKCNFKENADYNAALNISNPKLKSTKEEP

SEQ ID NO: 566 - protein, 726 aa, synthetic construct
SEVEFSHEYWMRHALTLAKRARDEREVPVGAILVLNNRVIGEGWNRAIGLHDPTAHAEIMALRQGGLVMQNYRLIDATLYVTFEPCVMCAGAMIHSRIGRVVFGVRNSKHGAAGSLVNVLNYPGMNHRVEITEGILADECAALLCDFYRMPRQVFNARKKARSNINSGGSSGGSSGSETPGTSESPTPESSGGSPGGSAKNTITKTLKLRIVRPYNSAEVEKIVADEKNNREKIALEKNKDKVKEACSKHLKVAAYCTTQVERNACLFCKARKLDDKFYQKLRGQFPDAVFWQELGGIFRQLQKQAAEIYNQSLIELYYEIFIKGKGITNASRVEHYLSDVCYTRAAELFKNAAIASGLRSKVRSNFRLKELKNMKSGLPTTKSDNFPIPLVKQKGGQYTGFEISSHNSDFIIKIPFGRWQEKEEIDKYRPWEKFDFEQVRKSPKPISLLLSTQRRKKNKGWSKDEGTEAEIRRVMNGDYQTSYIEVKRGSKIGEKSAWMLNLSIDVPKIDKGVDPSIIGGIDVGVKSPLVCAINNAFSRYSISDNDLFHFNKKMFARRRILLKKNRHRRAGHGAKNKLKPISILTGKSERFRKKLIERWACEIADFFIKNKVGTVQMENLESMKRKEDSYFNIRLRGFWPYAEMQNKIEYKLKQYGIEIRRVAPNNTSRTCSKCGHLNNYFNFEYRRKYKFPHFKCEKCNFKEDADYNAALNISNPKLKSTKEEP

SEQ ID NO: 567 - protein, 726 aa, synthetic construct
SEVEFSHEYWMRHALTLAKRARDEREVPVGAVLVLNNRVIGEGWNRAIGLHDPTAHAEIMALRQGGLVMQNYRLTDATLYVTFEPCVMCAGAMIHSRIGRVVFGVRNSKRGAAGSLMNVLNYPGMNHYVEITEGILVDECAALLCDFYRMPRQVLNAQKKAQSSINSGGSSGGSSGSETPGASESVTPKSSVGSSAGSTKNTITKTLKLRIVRPYNSAEVEKIVTDEKNNREKIALEKNKDKVKEACSKHLKMASYCTTQVERNACLFCKARKLDDKFYQKLRGQFPDAVFWQELGGIFRQLQKQAAEIYNQSLIELYYEIFIKGKGITNASRVEHYLSDVCYTRAAELFKNAAIASGLRSKVRSNFRLKELKNMKSGLPTTKSDNFPIPLVKQKGGQYTGFEISSHNSDFIIKIPFGRWQVKEEIDKYRPWEKFDFEQVRKSPKPISLLLSTQRRKKNKGWSKDEGTEAEIRRVMNGDYQTSYIEVKRGSKIGEKSAWMLNLSIDVPKIDKGVDPSIIGGIDVGVKSPLVCAINNAHSRYSISDNDLFHFNKKMFARRRILLKKNRHKRAGHGAKNKLKPITILTEKSGRFRKKLIERWACEIANFFIKNKVGTVQMENLESMKRKEDSYFNIRLRGFWPYAEMQNKIEFKLKQYGIKIRRVAPNNTSKTCSKCGHLNNYFSFEYRKKNKFPHFKCEKCNFKEDADYNAALNISNPKLKNTREEP

SEQ ID NO: 568 - protein, 726 aa, synthetic construct
SEVEFSHEYWMRHALTLAKRARDEREVPVGAILVLNNRVIGVGWNRAIGLHDPTAHAEIMALRQGGLVMQNYRLIDATLYVTFEPCVMCAGAMIHSRIGRVVFGVRNSKHGAAGSLVNVLNYPGMNHRVEITEGILADECAALLCDFYRMPRQAFNARKKAQSSINSGGSSGGSSGSETPGTSESATPKSSGGSSGGSAKNTITKALKLRIVRPYNSAEVEKIVADEKNNRERIALEKNKDKVKEACSKHLKVAAYCTTQVERNACLFCKARELDDKFYQKLRGQFPDAVFWQEIGEIFRQLQKQAAEIYNQSLIELYYEIFIKGKGFANASSVEHYLSDVCYTRAAELFKNAAIASGLRGKVKSNFRLKELKNMRSGLPTTKSDNFPIPLVKQKGGQYAGFEISSHNDDFIIKIPFGRWQVKKEIDKYRPWEKFDFEQVRKSPKPISLLLSTRRRKRNKGWSKDEGTEAEIRKVMNGDYQTSYIEVKRGSKIGEKSAWMLNLSIDVPKIDKGVDPSIVGGIDVGVKSPLVCAIDNALSRYSISDNDLFHFNKKMFARRRILLKKNRHRRAGHGAKNKLKPISILTEKSKRFRKKLIERWACEIADFFIKNKVGTVQMENLESMKRKEDSYFNIRLRGFWPYAEMQNKIEFKLKQYGIEIRKVAPNNTSKTCSKCGHLNNYFNFEYRKKNKFPHFKCEKCNFKENADYNAALNISNPKLKSTKEGP

SEQ ID NO: 569 - protein, 726 aa, synthetic construct
SEVEFSHEYWMRHALTLARRARGEREVPVGAVLVLNNRVIGEGWNRAIGLHDPTAHAEIMALRQGGLVMQNYRLTDATLYVTFEPCVMCAGAMIHSRIGRVVFGVRNSKRGAAGSLMNVLNYPGMNHCVEITEGILVDECAALLCDFYRMPRQVLNAQKKAQSSISSGGSSGGSSGSETPGASESATPKSSGGSSAGSTKNTITKALKLRIVRPYNSAEVEKIVADEKNNRERIALEKNKDKVKEACSKHLKVAAYCTTQVERNACLFCKARKLDDKFYQKLRGQFPDAVFWQETGEIFRQLQRQAAEIYNQSLIELYYEIFIKGKGFANASSVEHYLSDVCYTRAAELFKNAAIASGLRGKVKGNFRLKELKNMKSGLPTTKSDNFPIPLVKQKGGQYTGFEISSHNDDFIIKIPFGRWQAKKEIDKYRPWEKFDFEQVRRSPKPISLLLSTQRRKRNKGWSKDEGTEAEIRKVMNGDYQTSYIEVKRGSKIGEKSAWMLNLSIDVPKIDKGVDPSIIGGIDVGVKSPLVCAINNAFSRYSISDNDLFHFNKKMFARRRILLKKNRHKRAGHGAKNKLKPISILTEKSKRFRKKLIERWACEIADFFIKNKVGTVQMENLESMKRKEDSYFNIRLRGFWPYAEMQNKIEFKLKQYGIEIRKVAPNNTSKTCSKCGHLNNYFNFEYRKKNKFPHFKCEKCYFKEDADYNAALNISNPKLRSTKEEP

SEQ ID NO: 570 - protein, 726 aa, synthetic construct
SEVEFSHEYWMRHALTLAKRARDEREVPVGAVLVLNNRVIGEGWNRAIGLHDPTAHAEIMALRQGGLVMQNYRLTDATLYVTFEPCVMCAGAMIHSRIGRVVFGVRNSKRGAAGSLMNVLNYPGMNHCVEITEGILVDECAALLCDFYRMPCQVLNARKKAQSSISSGGSSGGSSGSDTLGASESATPKSSVGSSASSTKNTITKTLKLRIVRPYNCAEVEKIVADEKNNRERIALEKNKDKVKEACSKHLKVAAYCTTQVERNACLFCKARKLDDKFYQKLRDQFPDAMFWQEIGEIFRQLQRQAAEIYNQSLIELYYEVFIKGKGFANASSVEHYLSDVCYTRAAELFKNAAIASGLRGKVKSNFRLKELKNMKSGLPTTKSDNFPIPLVRQKGGQYTGFEISSHNGDFIIKIPFGRWQAKKEIDKYRPWERFDFEQVRKSPKPISLLLSTQRRKRNKGWSKDEGTEAEIRKVMNGDYQTSYIEVKRGSKIGEKSAWMLNLSIDVPKIDKGVDPSIIGGIDVGVKSPLVCAINNAFSRYSISDNDLFRFNKKMFARRRILLKKNRHKRAGHGAKNKLKPISILTEKSKRFRKKLIERWACEIADFFIKNKVGTVQMENLESMKRREDSYFNIRLRGFWPYAEMQNKIEFKLRQYGIEIRKVAPNNTSKTCSKCGHLNNYFNFEYRKKNKFPHFKCEKCNFKENADYNAALNISNPKLKSTKEEP

SEQ ID NO: 571 - protein, 726 aa, synthetic construct
SEVEFSHEYWMRHALTLAKRARDEREVPVGAILVLNNRVIGEGWNRAIGLHDPTAHAEIMALRQGGLVMQNYRLIDATLYVTFEPCVMCAGAMVHSRIGRVVFGVRNSKRGAAGSLMNVLNYPGMNHCVEITEGILVDECAALLCDFYRMPRQVLNAQRKAQSSISSGGSSGGSSDSETPGTSESATPESSGGGSSGSAKDTITKTLQLRIVRPYNSAEVEKIVADEKNNREKIALEKNKDKVKEACSKHLKVASYCTTQVERNACPFCKARKLDDKFYQKLRGQFPDAVFWQELGEILRQLQKQAAEIYNQSLIELYYEIFIKGRGFANASSVEHYLSDVCYTRAAELFKNAAIASGLRGKVKGNFRLKELKNMKSGLPTTKSDNFPIPLVKQKGGQYTGFEISSHNDDFIIKIPFGRWQVKKEIDKYRPWEKFDFEQVRKSPKPISLLLSTQRRKRNKGWSKDEGTEAEIRKVMNGDYQTSYIEVKRGSRTGEKSAWMLNLSIDVPKIDKGVDPSIIGGIDVGVKSPLVCAINNAFSRYSISDNDLFRFNKKMFARRRILLKKNRHKRAGHGAKNKLKPITILTEKSRRFRKKLIERWACEIADFFIKNKVGTVQMENLEGMKRKEDSYFNIRLRGFWPYAEMQNKIEFKLKQYGIEIRKVAPNNTSKTCSKCGHLNNYFNFEYRKKNKFPHFKCEKCSFKENADYNAALNISNPKLKSTREEP

SEQ ID NO: 572 - protein, 726 aa, synthetic construct
SGVEFSHEYWMRHALTLAKRARDEREVPVGAVLVLNNRVIGEGWNRAIGLHDPAAHAEIMALRQGGLVMQNYRLIGATLYVTFEPCVMCAGAMIHSRVGRVVFGVRNNKHGAAGSLVNVLNYPGMNHRVEITEGILADECAALLCDFYRMPRQVFNARKKAQSGINPGGSSGGSSGSETPGTSESATPESSGGSSGGSAKNTITKTLQLRIVRPYNSAEVEKIVTDEKNNREKIALEKNKDKVKEACSKHLKMASYCTTQVERNACLFCKARKLDDKFYQKLRGQFPDAVFWQELGGIFRQLQKQAAEIYNQSLIELYYEIFIKGKGITNASRVEHYLSDVCYTRAAELFKNAAIASGLRSKVRSNFRLKELKNMKSGLPTTKSDNFPIPLVKQKGGQYTGFEISSHNDDFIIKIPFGRWQVKKEIDKYRPWEKFDFEQVRKSPKPISLLLSTQRRKRNKGWSKDEGTEAEIRKVMNGDYQTSYIEVKRGSKIGEKSAWMLNLSIDVPKIDKGVDPSIIGGIDVGVKSPLVCAINNALSRYSISDNDLFHFNKKMFARRRILLRKNRHKRAGHGAKNKLKPITIMTEKSKRFRKKLIERWACEIADFFIKNKVGTVQMENLESMKRREDSYFNIRLRGFWPYAEMQNKIEFKLKQYGIVVRKVAPNNTSKTCSKCGHLNNYFNFEYRKKNKFPHFKCEKCNFKEDADYNAALNISNPKLKSTKGEP

SEQ ID NO: 573 - protein, 726 aa, synthetic construct
SEVEFSHEYWMRHALTLAKRARDEREVPVGAVLVLNNRVIGEGWNRAIGLHDPTAHAEIMALRQGGLVTQNYRLIDATLYVTFEPCVMCAGAMIHSRIGRVVFGVRNSKHGAAGSLMNVLNYPGMNHRVEITEGILADECAAQLCDFYRMPRQVFNARKKAQSSINPGGSSGGSSGSETPGTSESATPVSSGGSSGGSAKNTITKTLKLRIVRPYNSAEVEKIVADEKNNREKIALEKNKDRVKEACSKHLKVAAYCTTQVERNACLFCKARRLDDKFYQKLRGQFPDAVFWQEIGEIFRQLQKQAAEIYNQGLVELYYEIFIKGKGIANASSVERYLSDVCYTRAAELFKNAAIASGLRNKIKSNFRLKELRNMKSGLPTTKSDNFPIPLVRQKGGQYTGFEISNHNGDFIIKIPFGRWQVKKEIDKYRPWEKFDFEQVRKSPKPISLLLSTQRRKRNRGWSKDEGTEAEIRKVMNGDYQTSYIEVKRGSKIGEKSAWMLSLSIDVPKIDKGVDPSIIGGIDVGVKSPLVCAINNAFSRYSISDNDLYRFNKKMFARRRILLGKNRHKRAGHGVKNKLKPITILTEKSGRFRKKLIERWACEIADFFVKNKVGTVQMENLESMKRKEDSYFNIRLRGFWPYAEMQNKIEFKLKQYGIKVRKVAPNNTSKTCSKCGHLNNYFSFEYRKKNKFPHFKCEKCNFKENADYNAALNISNPKLKSTKEEP

SEQ ID NO: 574 - protein, 726 aa, synthetic construct; identical to SEQ ID NO: 294

SEQ ID NO: 575 - protein, 726 aa, synthetic construct; identical to SEQ ID NO: 294

SEQ ID NO: 576 - protein, 726 aa, synthetic construct
SEVEFSHEYWMRHALTLAKRARDEREVPVGAVLVLNNRVIGEGWNRAIGLHDPTAHAEIMALRQGGLVMQNYRLTDATLYVTFEPCVMCAGAMIHSRIGRVVFGVRNSKRGAAGSLMNVLNYPGMNHCVEITEGILVDECAALLCDFYRMPRQVLNAQKKAQSSISSGGLSGGSSGSETPGASGSVTPKSSGGSSAGPTKDTITKTLKLRIVRPYNSAVVEKIVADEKNSREKIALEKNKDKVKEACSEHLKVAAYCTTRVERNACLFCKARKLDDGFYQKLRGQFPDAVFWQEIGEIFRQLQKQAAEIYNQSLIELYYEIFIKGKGFANASSVEHYLSDVCYTRAAELFKNAAIASGLRGKVKSNFRLKELKNMKSGLPTTKSDNFPIPLVKQKGGQYTGFEISNHNGDFIIKIPFGRWQVKKEISKHRPWEKFDFEQVRKSPKPISLLLSTQRRKRNKGWSKDEGTEAEIRKVMNGDYQTSYIEVKRGSKTGEKSAWMLNLSIDVPKIDKGVDPSIIGGIDVGVKSPLVCAINNALSRYSISDNDLFRFNKKMFARRRILLKKNRHKRAGHGARNKLKPITVLTEKSERFREKLIERWACEIANFFIKNKVGTVQMENLESMKRREDGYFNIRLRGFWPYAEMQSKIEFKLKQYGIEIRKVAPNNTSKTCSKCGHLNNYFNFEYRKKNKFPHFKCEKCNFKEDADYNAALNISNPKLKSTKEEP

SEQ ID NO: 577 - protein, 726 aa, synthetic construct
SEVEFSHEYWMRHALTLAKRARDEREVPVGAILVLNNRVIGEGWNRAVGLHDPTAHAEIMALRQGGLVMQNYRLIEATLYVTFEPCIMCAGAMIHSRIGRVVFGVRNSKRGAAGSLMNVLNYPGMNHRVEITEGILVDECAALLCDFYRMPRQVLNAQKKAQSSISPGGSSGGCSGSEMPGASESVTPKSSGGSSAGSTKNTITKTLKLRIVRPYNSAEVEKIVADEKNSREKIALERNKDKVKEACSEHLKVASYCTTQVERNACLFCKARKLDDKFYQRLRGQFPDAVFWQELGEIFRQLQKQAAEIYNQSLIELYYEIFIKGKGFANASSVEHYLSDVCYTRAAELFKNAAIASGLRGKVKSNFRLKELKNMKSGLPTTKSDNFPIPLVRQKGGQYTGFEISNHNGDFIIKIPFGRWQVKKEICKHRPWEKFDFEQVRKNPKPISLLLSTQRRKRNKGWGKDEGTEAEIKKVMNGDYQTSYIEVKRGSKIGEKNAWMLNLSIDVPKIDKGVDPSIIGGIDVGVKSPLVCAINNALSRYSISDNDLFHFNKKMFARRRILLRKNRHKRAGHGARNKLKPISILTEKSKRFRKKLIERWACEIADFFIKNKVGTVQMENLESMKRKEDSYFNIRLRGFWPYAEMQNKIEFKLKQYGIEIRKVAPNNTSKTCSKCGHLNNYFSFEYRKKNKFPHFKCEKCNFKENADYNAALNISNPKLKSTKEEP

SEQ ID NO: 578 - protein, 726 aa, synthetic construct
SEVEFSHEYWMRHALTLAKRARDEREVPVGAILVLNNRVIGEGWNRAIGLHDPTAHAEIMALRQGSLVIQNYRLIDATLYVTFEPCVMCAGAMIHSRIGRVVFGVRNSKHGAAGSLVNVLNYPGMNHRVEITEGILADECAALLCDFYRMPRRVFNARMKAQSSISPGGSSGGSSGSETPGTSESATPESSGGSSGGSAKNTITKTLKLRIVRPYNSAEVEKIVADEKNNREKIALEKNKDRVKEACSKHLKVASYCTTQVERNACLFCKARKLDDKFYQKLRDQFPDAVFWQELGEILRQLQKQAAEIYNQSLIELYYEIFIKGKGFANASSVEHYLSDVCYTRAAELFKNAAIASGLRGKVKSNFRLKELKNMKSGLPTTKSDNFPVPLVKQKGGQYTGFEISNHNSDFIIKIPFGRWQVKEEINKYRPWEKFDFEQVRKSPKPISLLLSTQRRKRNRGWSKDEGTEAEIRKVMNGDYQTSYIEVKRGSKIGEKSAWMLNLSIDVPKIDKGVDPSITGGIDVGVKSPLVCAINNAFSRYSISDNDLFRFNKKMFARRRILLGKNRHKRAGHGVKNKLKPITILTEKSGRFRKKLIERWACEIADFFVKNKVGTVQMENLESMKRKEDSYFNIRLRGFWPYAAMQNKIEFKLKQYGIKVRKVAPNNTSKTCSKCGHLNNYFNFEFRKKNKFPHFKCEKCNFKEDADYNAALNISNPKQKSTKEEP

SEQ ID NO: 579 - protein, 726 aa, synthetic construct
SEVEFSHEYWMRHALSLAKRARDEREVPVGAVLVLNNRIIGEGWNRAIGLHDPTAHAEIMALRQGGLVMQNYRLTDATLYVTFEPCVMCAGAMVHSRIGRVVFGVRNSKRGAAGSLMNVLNYPGVNHCVEITEGILVDECAALLCDFYRMPRQVLNAQKKAQSSISSGGSSGGCSGSEMPGASESVTPKSSGGSSAGSTKNTITKTLKLRIVRPYNSAEVEKIVADEKNSREKIALERNKDKVKEACSEHLKVAAYCTTQVERNACLFCKARKLDDRFYQKLRGQFPDAVFWQETGEIFRQLQRQAAEIYNQSLIELYYEIFIKGKGFANASSVEHYLSDVCYTRAAELFKNAAIASGLRGKVKSNFRLKELKNMKSGLPTTKSDNFPIPLVKQKGGQYTGFEISSHNDDFIIKIPFGRWQMKKEIDRYRPWEKFDFEQVRRSPKPISLLLSTQRRKRNKGWSKDEGTEAEIRKVMNGDYQTSYIEVKRGSKIGEKSAWMLSLSIDVPKIDKGVDPSIIGGIDVGVKSPLVCAINNAFSRYSISDNDLFRFNKKMFARRRILLKKNRHKRAGHGARNKLKPITVLTEKSERFRKKLIERWACEIANFFIKNKVGTVQMENLESMKRREDSYFNIRLRGFWPYAEMQSKIEFKLKQYGIKIRKVAPNNTSKTCSKCGHLNNYFNFEFRKKNKFPHFKCEKCNFKEDADYNASLNISNPKLKSTKEEP

SEQ ID NO: 580 - protein, 726 aa, synthetic construct
SEVEFSHEYWMRRALTLAKRARDEREVPVGAVLVLNNRVIGVGWNRAVGLHDPTAHAEIMALRQGGLVMQNYRLIEATLYVTFEPCIMCAGAMIHSRIGRVVFGVRNSKRGAAGSLMNVLNYPGMNHRVEITEGILADECTALLCDYYRMPRQVFNARKKAQSSINSGGSSDGGSGSETPGTSESATPESSGGSSGGSAKNTITKTLKLRIVRPYNSAEVEKIVADEKNNREKIALEKNKDKVKEACSEHLKVAAYCTTQVERSACLFCKARKLDDKFYQKLRGQFPDAVFWQEIGEIFRQLQKQAAEIYNQSLIELYYEIFIKGKGFANASSVEHYLSDVCYTRAAELFKNAAIASGLRGKVKSNFRLKELKNMRSGLPTTKSDNFPIPLVKQKGGQYTGFEISSHNDDFIIKIPFGRWQVKKEIDKYRPWEKFDFEQVRKSPKPISLLLSTQRRKRNKGWSKDEGTEAEIRKVMNGDYRTSYIEVKRGSKTGEKSAWVLNLSIDVPKIDKGVDPSIIGGIDVGVKSPLVCAINNAFSRYSISDNDLFRFNKKMFARRRILLKKSRHKRAGHGAKNKLKPITILTEKSGRFRKKLIERWACEIADFFIKNKVGTVQMENLESMKRKEDSYFNIRLRGFWPYAEMQNKIEFKLKQYGIKIRKVAPNNTSKTCSKCGHLNNYFSFEYRKKNKFPHFKCEKCNFKEDADYNAALNISNPKLKSTKEEP

SEQ ID NO: 581 - protein, 726 aa, synthetic construct
SEVEFSHEYWMRHALTLAKRARDEREVPVGAVLVLNNRVIGEGWNRAIGLHDPTAHAEIMALRQGGLVMQNYRLIDATLYVTFEPCVMCAGAMIHSRIGRVVFGVRNSKHGAAGSLMNVLNYPGMNHRVEITEGILADECAALLCDFYRMPRQVFNARKKAQSSINPGGPSGGSSGSETPDTSESVTPKSSGGSSAGSTKNTITKTLKLRIVRPYNSAEVEKIVADEKNSREKIALEKNKGKVKEACSKHLKVASYCTTQVERNACPFCKARKLDDKFYQKLRGQFPDAVFWQELGGILRQLQKQAAEIYNQSLIELYYEIFIKGRGFANASSVEHYLSDVCYTRAAELFKNAAIASGLRGKVKSNFRLKELKNMKSGLPTTKSDNFPIPLVRQKGGQYTGFEISSHNDDFVIKIPFGRWQVKKEIDKYRPWEKFDFEQVRKSPKPISLLLSTQRRKRNKGWSKDEGTEAEIRKVMNGDYQTSYIEVKRGSKIGEKSVWMLNLSIDVPKIDKGVDPSIIGGIDVGVKSPLVCAINNAFSRYSISDNDLFHFNKKMFARRRILLKKNRHRRAGHGARNKLKPITVLTEKSKRFRKKLIERWACEIANFFIKNKVGTVQMENLESMKRKEDSYFNIRLRGFWPYAEMQNKIEFKLKQYGIVVRKVAPNNTSKTCSQCGHLNNYFNFEYRKKNKFPYFKCEKCNFKENADYNAALNISNPQLKSTKGEP

SEQ ID NO: 582 - protein, 726 aa, synthetic construct
SEVEFSHEYWMRHALTLAKRARDEREVPVGAILVLNNRVIGEGWNRAIGLHDPTAHAEIMALRQGGLVMQNYRLIDATLYVTFEPCVMCAGAMIHSRIGRVVFGVRNNKHGAAGSLVNVLNYPGMNHRVEITEGILVDECAALLCDFYRMPRQVFNAQKKAQSTINSGGSSGGSSGSETPGTSESPTPESSGGSSGGSTKNTITKTLKLRIVRPYNSAEVEKIVADEKNNRERIALEKNKDKVKEACSKHLKVAAYCTTQVERNACPFCKARKLDDKFYQKLRGQFPEAVFWQEIGEIFRQLQKQAAEIYNQSLIELYYEIFIKGKGFANASSVEHYLSDVCYTRAAELFKNAAIASGLRGKVKSNFRLKELKNMRSGLPTTKSDNFPIPLVKQKGGQYTGFEISSHNDDFIIKIPFGRWQMKKEIDRYRPWEKFDFEQVRKSPKPISLLLSTQRRKRNKGWGKDAGTEAEIRKVMNGDYQTSYIEVKRGSKIGEKSAWMLNLSIDVPKIDKGVDPGIIGGIDVGVKSPLVCAINNASSRYSISDNDLFRFNKKMFARRRILLKKSKHKRAGHGAKNKLKPITILTEKSRRFRKKLIERWACEIADFFIKNKVGTVQMENLESMKRKEDSYFNIRLRGFWPYAEMQNKIEFKLKQYGIVIRKVAPNNTSRTCSKCGHLNNYFNFEYRKKNKFPHFKCEKCNFKEDADYNAALNISNPKLKSTKEES

SEQ ID NO: 583 - protein, 726 aa, synthetic construct
SEVELSHEYWMRHALTLAKRARDGREVPVGAVLVLNNRVIGEGWNRAIGLHDPTAHAEIMALRQGGLVMQNYRLIDATLYVTFEPCVMCAGAMVHSRIGRVVFGVRNSKRGAAGSLMNVLDYPGMNHRVEITEGILADECAALLCDFYRMPHRVFNGRKKAQSSINPGGSSGGSSGSKTPGTSESATPGSSGGGSSGSAKNTITKTLQLRIVRPYNSAEVEKIVADEKNNREKIALEKNKDKVKEACSKHLKVASYCTTQVERNACPFCKARKLDDKFYQKLRGQFPDAVFWQEIGEIFRQLQRQAAEIYNQSLIELYYEIFIKGKGFANASSVEHYLSDVCYTRAAELFKNAAIASGLRGKVKSNFRLKELKNMKSGLPTTKSDNFPIPLVKQKGGQYTGFEISSHNDDFIIKIPFGRWQVKKEIDKYRPWEKFDFEQVRKSPKPISLLLSTQRRKRNKGWSKDEGTEAEIRKVMNGDYQTSYIEVKRGSKVGEKSAWMLSLSIDVPKIDKGVDPSIIGGIDVGVRSPLVCAINNAFSRYSISDNDLFHFNKKMFARRRILLKKNRHRRAGHGAKNKLKPITVLTEKSKRFRKKLIERWACEIANFFIKNKVGTVQMENLESMKRREDSYFNTRLRGFWPYAEMQNKIEFKLKQYGIEIRKVAPNNTSKTCSKCGHLNNYFNFEYRKKNKFPHFKCEKCNFKENADYNAALNISNPRLKSTKEEP

SEQ ID NO: 584 - protein, 726 aa, synthetic construct
GEVEFSHEYWMRRALTLAKRARDEREVPVGAILVLNNRVIGEGWNRAIGLHDPTAHAEITALRQGGLVMQNYRLIDATLYVTFEPCVMCAGAMIHSRIGRVVFGVRNSKHGAAGSLVNVLNYPGMNHRVEITEGILADECAALLCDFYRMPRQVFNARKKAQPSINPGGSSGGSSGSETPGTSESATPESSGGNSGGSAKNTITKTLTLRIVRPYNSAEVEKIVADEKNNREKIALEKNKDKVKEACSEHLKVATYCTTRVERNACPFCKARKLDDKFYQKLRGQFPDAVFWQEISEIFRQLQKQAAEIYNQSLIELYYEIFIKGKGFANASSVEHYLSDVCYTRAAELFKNAAIASGLRGKVKSNFRLKELKNMKSGLPTTKSDNFPIPLVKQKGGQYTGFEISSHNDDFIIKIPFGRWQVKKEIDKYRPWEKFDFEQVRKSPKPISLLLSTQRRKRNKGWSKDEGTEAEIRKVMNGDYQTSYIEVKRGSKIGEKSAWMLSLSIDVPKIDKGVDPSIIGGIDVGVKSPLVCAINNAFGRYCISDNDLFRFNKKMFARRRILLKRNRHKRAGHGARNKLKPITVLTEKSKRFRKKLIERWACEIADFFIKNKVGTVQMENLESMKRKEDSYFNIRLRGFWPYAEMQNKIEFKLKQYGIVVRKVAPDNTSKTCSKCGHLNNYFSFEYRKKNKFPHFKCEKCSFKENADYNAALNISNPKLKSTKEEP

SEQ ID NO: 585 - protein, 726 aa, synthetic construct
SEVEFSHEYWMRHALTLAKRARDEREVPVGAVLVLNNRVIGEGWNRAIGLHDPTAHAEIMALRQGGLVMQNYRLVDATLYVTFEPCVLCAGAMVHSRIGRVVFGVRNSKRGAAGSLMNVLNYPGMNHRVEITEGILADECAALLCDFYRMPRQVFNARKKARSNINSGGSSGGNSGSETPGTSESATPESSGGSSGGSAKNTITKTLKLRIVRPYNSAEVEKIVADEKSNREKIALEKNKDKVKEACSKHLKVASYCTTQVERNACLFCKARKLDDKFYQKLRGQFPDAVFWQEIGEIFRQLQKQAAEIYNQSLIELYYEIFIKGKGFANASSVEHYLSDVCYTRAAELFKNAAIASGLRGKVKSNFRLKELKNMKSGLPTTKSDNFPIPLVKQKGGQYTGFEISSHNDDFIIKIPFGRWQVKEEVDKYRPWEKFDFEQVRKNPKPISLLLSTQRRKRNKGWSKDEGTEAEIRKVMNGDYQTSYIEVKRGSKIGEKSAWMLNLSIDVPKIDKGVDPSIIGGIDVGVKSPLVCAINNAFSRYSISDNDLFRFNKKVFARRRILLKKNRHKRAGHGTKNKLKPITILTEKSGRFRKKLIERWACEIANFFIKNKVGTVQMENLESMKRKEDSYFNIRLRGFWPYAEMQNKIEFKLKQYGIKIRKVAPNNTSKTCSKCGHLNNYFSFEYRKKNKFPHFMCEKCNFKEDADYNAALNISNPKLKSTKEEP

SEQ ID NO: 586 - protein, 726 aa, synthetic construct
SEVEFSHEYWMRHALTLAKRARDEREVPVGAILVLNNRVIGEGWNRAIGLHDPTAHAEIMALRQGGLVMQNYRLVDATLYVTFEPCVMCAGAMIHSRVGRVVFGVRNSKHGAAGSLMNVLNYPGMNHRVEITEGILADECAALLCDFYRMPRRVFNARKKAQSSINPGGSSGGSSGSEAPGTSESATPESSGGSSGGSAKNTITKTLKLRIVRPYNSAEVEKIVADEKNNREKIALEKNKDKVKEACSKHLKVAAYCTTQVERNACLFCKARRLDDKFYQKLRGQFPDAVFWQEIGEIFRQLQKQAAETYNQSLIELYYEIFIKGKGIASASRVEHYLSDVCYTRAAELFKNAAIASGLRGKVKSNFRLKELKNMKSGLPTTKSDNFPIPLVKQKGGQYTGFEISSHNDDFIIKIPFGRWQVKKEIDKYRPWEKFDFEQVRKSPKPISLLLSTQRRKRNKGWNKDEGTEAEIRKVMNGDYQTSYIEVKRGSKIGEKSAWMLNLSIDVPKIDKGVDPSIIGGIDVGVKSPLVCAINNAFSRFSISDNDLFRFNKKMFARRRILLKKNRHKRAGHGAKNKLKPITILTEKSGRFRKKLIERWACEIADFFIKNKVGTVQMENLESMKRKEDSYFNIRLRGYWPYAEMQNKIEFKLKQYGIKVRKVAPNNTSKTCSKCGHLNNYFSFEYRKKNKFPHFKCEKCNFKENADYNAALNISNPKLKSTKEEP

SEQ ID NO: 587 - protein, 726 aa, synthetic construct
SEVEFSHEYWMRRALTLAKRARDEREVPVGAVLVLNNRVIGVGWNRAVGLHDPTAHAEIMALRQGGLVMQNYRLIEATLYVTFEPCIMCAGAMIHSRIGRVVFGVRNSKRGAAGSLMNVLNYPGMNHRVEITEGILADECAALLCDYYRMPRQVFNARKKAQSSINSGGSSDGGSGSETPGTSESATPESSGGSSGGSAKNTITKTLKLRIVRPYNSAEVEKIVADEKSNREKIALEKNKDKVKEACSKHLKMASYCTTQVERNACLFCKARKLDDKFYQKLRGQFPDAVFWQELGGIFRQLQKQAAEIYNQSLIELYYEIFIKGKGITNASRVEHYLSDVCYTRAAELFKNAAIASGLRSKVRSNFRLKELKNMKSGLPTTKSDNFPIPLVKQKGGQYTGFEISSHNSDFIIKIPFGRWQVKEEIDKYRPWEKFDFEQVRKSPKPISLLLSTQRRKKNKGWGKDEGTEAEIRRVMNGDYQTSYIEVKRGSKIGEKSAWMLNLSIDVPKIDKGVDPSIIGGIDVGVISPLVCAINNAFSRYSISDNDLFHFNKKMFARRRILLKKNRRRRAGHGAKNKLKPITIMTEKSKRFRKKLIERWACEIADFFIKNRVGTVQMENLESMKKKEDSYFNIRLRGFWPYAEMQNKIEFKLKQYGIVVRKVAPNNTSKTCSKCGHLNNYFNFEYRKKNKFPHFKCEKCNFKEDADYNAALNISNPKLKSTRGEP

SEQ ID NO: 588 - protein, 726 aa, synthetic construct
SEDEFSHEYWMRHALALARHARDEGEVPVGAVLVLNNRVIGEGWNRAIGLHDPTAHAEIMALRQGGLVMQNHRLVNATLYVTFEPCVMCAGAMIHSRIGRVVFGVRNSKRGAAGSLMNVLNYPGMNHCVEITEGILVDECAALLCDFYRMPRQVLNAQKKAQSSISSGGSSGGSSGSETPGASGSVTPKSSGGSSAGSTKDTITKTLQLRIVRPYNSAEVEKIVTDEKNNREKIALEKNKDKVKEACSKHLKMAAYCTTQVERNACLFCKARKLDDRFYQKLRGQFPDAVFWQEIGEIFRQLQKQAAEIYNQSLIELYYEIFIKGKGFAIASSVEHYLSCVCYTRAAELFKNAAIASGLRGKVKSNFRLKELKNMKSGLPTTKSDNFPIPLVKQKGGQYTGFEISSHNDDFIIKIPFGRWQVKEEIDKYRPWEKFDFEQVRKNPKPISLLLSTQRRKRNKGWSKDEGTEAEIRKVMNGDYQTSYIEVKRGSKIGEKSAWMLNLSIDVPKIDKGVDPSIIGGIDVGVKSPLVCAINNAFSRYSISDNDLFRFNKKVFARRRILLKKNRHKRAGHGTKNKLKPITILTEKSGRFRKKLIERWACEIANFFIKNKVGTVQMENLESMKRKGDSYFNIRLRGFWPYAEMQNKIEFKLKQYGIKIRKVAPNNTSKTCSKCGHLNNYFSFEYRKKNKFPHFKCEKCNFKEDADYNAALNISNPRLKSTKEEP

SEQ ID NO: 589 - protein, 726 aa, synthetic construct
SEVEFSHEYWMRHALTLAKRARDEREVPVGAVLVLNNRVIGEGWNRAIGLHDPTAHAEIMALRQGGLVMQNYRLIDATLYVTFEPCVMCAGAMIHSRIGRVVFGVRNSKHGAAGSLVNVLNYPGMNHRVEITEGILADECAALLCDFYRMPRQVFNARKKAQSSISSGGSSGGSSGSETPGASGSVTPKSSGGSSAGSTKDTITKTLKLRIVRPYNSAEVEKVVADEKNNREKIAIEKNKDMVKEACSKHLKVASYCTTQVERNACLFCKARKLDDKFYQKLRGQFPDAVFWQELGGIFRQLQKQAAEIYNQSLIELYYEIFIKGKGITNASRVEHYLSDVCYTRAAELFKNAAIASGLRSKVRSNFRLKELKNMKSGLPTTKSDNFPIPLVKQKGGQYTGFEISSHNSDFIIKIPFGRWQEKEEIGKYRPWEKFDFEQVRRSPKPISLLLSTQRRKKNKGWSKDEGTEAEIRRVMNGDYQTSYIEVKRGSKIGEKSAWMLNLSIDVPKIDKGVDPSIIGGIDVGVKSPLVCAINDAFSRYSISDNDLFHFNKKMFARRRILLKKNRRRRAGHGAKNKLKPITILTEKSVRFRKKLIERWACEIADFFIKNKVGTVQMENLESMKRKEDSYFNIRLRGFWPYAEMQNKIEFKLKQYGIEIRRVAPNNTSRTCSKCGHLNDYFNFEYRRKYKFPHFKCEKCNFKEDADYNAALNISNPKLKSTKEEP

SEQ ID NO: 590 - protein, 726 aa, synthetic construct
SEVEFSHEYWMRHALTLAKRARDEREVPVGAVLVLNNRAIGEGWNRAIGLHDPTAHAEIMALRQGGLVMQNYRLTDATLYVTFEPCVMCAGAMIHSRIGRVVFGVRNSKRGAAGSLMNVLNYPGMNHCVEITEGILVDECAALLCDFYRMPRQVLNAQKKAQSSINSGSSSGGSSGSETPGASGSVTPKSSGGSSAGSTKDTITKTLKLRIVRPYNSAEVEKIVADEKNSREKIALEKNKDKVKEACSEHLKVAAYCTTQVERNACLFCRARKLDDKFYLKLRDQFPDAVFWQEISEIFRQLQKQAAEIYNQSLIELYYEIFIKGKGIASTSRVGHYLSDVCYTRAAELFKNAAIASGLRGKVKSNFRLKELRNMKSGLPTTKSDNFPIPLVRQKGGQYTGFEISSHNDDFIIKIPFGRWQAKKEIDKYRPWEKFDFEQVRKSPKPISLLLSTQRRKRNKGWSKDEGTEAEIRKVMNGDYQTSYIEVKRGSKIGEKSAWMLNLSIDVPKIDKGVDPSIIGGIDVGVKSPLVCAINNASSRYSISDNDLFRFNKKMFARRRILLKKNRHKRAGHGAKNKLKPISILTGKSERFRKKLIERWACEIADFFIKNKVGTVQMENLESMKRKEDSYFNIRLRGFWPYAEMQNKIEFKLRQYGIEIRKVAPNNTSKTCSKCGHLNNYFDFEYRRKNKFPLFKCEKCSFKENADYNAALNISNPKLKSTKGEP

SEQ ID NO: 591 - protein, 726 aa, synthetic construct
SEVEFSHEYWMRRALTLAKRARDEREVPVGAVLVLNNRVIGVGWNRAVGLHDPTAHAEIMALRQGGLVMQNYRLIEATLYVTFEPCIMCAGAMIHSRIGRVVFGVRNSKRGAAGSLMNVLNHPGMNHRVEITEGILADECAALLCDYYRMPRQVFNARKKAQSSINSGGSSDGGSGSETPGTSESATPESSGGSSGGSAKNTITKTLKLRIVRPYNSAEVEKIVADEKNDREKIALEKNKDKVKEACSEHLKVAAYCTTQVERSACLFCKARKLDDKFYQKLRGQFPDAVFWQEIGEIFRQLQKQAAEIYNQSLIELYYEIFIKGKGFANASSVEHYLSDVCYTRAAELFKNAAIASGLRGKVKSNFRLKELKNMKSGLPTTKSDNFPIPLVKQKGGQYTGFEISSHNDDFIIKIPFGRWQVKKEIDKYRPWEKFDFEQVRKSPKPISLLLSTQRRKRNRGWSKDEGTEAEIRRVMNGDYQTSYIEVKRGSKIGEKSAWMLNLSIDVPKIDKGVDPSIIGGIDVGVKSPLVCAINNAFSRYSISDNDLFRFNKKMFARRRILLEKNRHKRAGHGVKNKLKPITILTEKSGRFRKKLIERWACEIADFFVKNKVGTVQMENLESMKRKEDSYFNIRLRGFWPYAEMQNKIEFKLKQYGIRVRKVAPNNTSKTCSKCGHLNNYFSFEYRKKNKFPHFKCEKCNFKENADYNAALNISNPKLKSTKEEP

SEQ ID NO: 592 - protein, 726 aa, synthetic construct
SEVEFSHEYWMRHALTLAKRARDEREVPVGAVLVLNNRVIGVGWNRAVGLHDPTAHAEIMALRQGGLVTQNYRLVDATLYVTFEPCVMCAGAMIHSRIGRVVFGVRNGKRGAAGSLMNVLNYPGMNHRVEITEGILADECAALLCDFYRMPRQVFNAQKKAQSNINPGGSSGGSSGSETPGTSESPTPESSGGSPGGSAKNTITKTLQLRIVRPYNSAEVEKIVADEKNNREKIALEKNKGKVKEACSKHLKVASYCTTQVERNACPFCKARKLDDKFYQKLRGQFPDAVSWQELGEILRQLQKQAAEIYNQSLIELYYEIFIKGRGFANAGSVEHYLSDVCYTRAAELFKNAAIASGLRGKVKSNFRLKELKNMKSGLPTTKSDNFPIPLVKQKGGQYTGFEISSHNDDFIIKIPFGRWQVRKEIDKYRPWEKFDFEQVRKNPKPISLLLSTQRRRRNKGWSKDEGTEAEIRKVMNGDYQTSYIEVKRGSKIGEKSAWMLNLSIDVPKIDKGVDPSIIGGIDVGVKSPLVCAINNAFSRYSISDNDLFRFNKKVFARRRILLKKNRHKRAGHGTKNKLKPITILTEKSGRFRKKLIERWACEIADFFIKNKVGTVQMENLESMKRKEDSYFNIRLRGFWPYAEMQNKIEFKLRQYGIKIRKVAPNNTSKTCSKCGHLNNYFSFEYRKKNKFPHFKCEKCNFKEDADYNAALNISNPKLKSTKEEP

SEQ ID NO: 593 - protein, 726 aa, synthetic construct
SEVEFSHEYWMRHALTLAKRARDEREVPVGAVLVLNNRAIGEGWNRAIGLHDPTAHAEIMALRQGGLVMQNYRLTDATLYVTFEPCVMCAGAMIHSRIGRVVFGVRNSKRGAAGSLMNVLNYPGMNHCVEITEGILVDECAALLCDFYRMPRQVLNAQKKAQSSISSGGSSGGSSGSETPGASGSVTPKSSGGSSAGSTKDTITKTLKLRIVRPYNSAEVEKVVADEKNNREKIAIEKNKDMVKEACSKHLKVASYCTTQVERNACLFCKARKLDDKFYQKLRGQFPDAVFWQELGGIFRQLQKQAAEIYNQSLIELYYEIFIKGKGITNASRVEHYLSDVCYTRAAELFKNAAIASGLRSKVRSNFRLKELKNMKSGLPTTKSDNFPIPLVKQKGGQYTGFEISSHNSDFIIKIPFGRWQEKEEIGKYRPWEKFDFEQVRRSPKPISLLLSTQRRKKNKGWSKDEGTEAEIRRVMNGDYQTSYIEVKRGSKIGEKSAWMLNLSIDVPKIDKGVDPSIIGGIDVGVKSPLVCAVNNAFSRYSISDNDLFRFNKKMFARRRILLGKNRHKRAGHGVKNKLKPITILTEKSGRFRKKLIERWACEIADFFVKNKVGTVQMENLESMKRKEDSYFNIRLRGFWPYAEMQNKIEFKLKQYGIKVRKVAPNNTSKTCSKCGHLNNYFSFEYRKKNKFPHFKCEKCNFRENADYNAALNISNPKLKSTKEEP

SEQ ID NO: 594 - protein, 726 aa, synthetic construct
SEVEFSHEYWMRHALTLAKRARDEREVPVGAVLVLNNRVIGVGWNRAIGLHDPTAHAEIMALRQGGLVTQNYRLINATLYVTFEPCVMCAGAMIHSRIGRVVFGVRNSKHGAAGSLVNVLNYPGMNHRVEITEGILADECAALLCDFYRMPRQVFNAQKKARPNINSGGSSGGRSGSETPGTSESATPESSGGSSGGSAKNTITKTLKLRIVRPYNSAEVEKIVADEKNSREKIALEKNKDKVKEACSEHLKVAAYCTTQVERNACLFCKARKLDDGFYQKLRGQFPDAVFWQELGEIFRQLQKQAAEIYNQSLIELYYEILIKGKGIANASRVEHYLSDVCYTRAAELFKNAAIASGLRSKIKSNFRLKELRNMKSGLPTTKSDNFPIPLVKQKGGQCTGFEISNHNSDFIIKIPFGRWQVKKEIDKYRPWEKFDFEQVRKSPKPISLLLSTQRRRRNKGWGKDEGTEAEIRKVMNGDYQTSYIEVKRGSRIGEKSAWMLSLSIDVPKIDRGVDPSIIGGIDVGVKSPLVCAINNALSRYSISDNDLFHFNKKMFARRRILLKKNRHRRAGHGARNKLKPITVLTEKSKRFRKKLIERWACEIANFFVKNKVGTVQMENLESMKRKEDSYFNIRLRGLWPYAEMQNKIEFKLKQYGIEVRKVAPNNTSKTCSKCGHLNNYFNFEYRKKNKFPHFKCEKCNFKENADYNAALNISNPKLKSTKEEP

SEQ ID NO: 595 - protein, 726 aa, synthetic construct
SEVEFSHEYWMRHALTLAKRARDEREVPVGAVLVLNNRVIGEGWNRAIGLHDPTAHAEIMALRQGGLVMQNYRLVDATLYVTFEPCVLCAGAMVHSRIGRVVFGVRNSKRGAAGSLMNVLNYPGMNHRVEITEGILADECAALLCDFYRMPRQVLNTQKKAQSSINSGDSSGGSSCGETPGTSESTTPESSGGSFGGSTKNTITKTLKLRIVRPYNSAEVEKIVADEKNNREKIALEKNKDKVKEACSKHLKVAAYCTTQVERNACLFCKARKLDDKFYQKLRGQFPDAVFWQEIGEIFRQLQKQAAEIYNQSLIELYYEIFIKGKGFANASSVEHYLSDVCYTRAAELFKNAAIASGLRGKVKSNFRLKELKNMRSGLPTTKSDNFPIPLVKQKGGQYTGFEISSHNDDFIIKIPFGRWQVKKEIDKYRPWEKFDFEQVRKSPKPISLLLSTQRRKRNKGWSKDEGTEAEIRKVLNGDYQTSYIEVKRGCKIGEKSAWMLNLCIDVPKIDKGVDPSIIGGIDVGVKSPLVCAINNAFSRYSISDNDLFHFNKKVFARRRILLKKNRHRRAGHGAKNKLKPITILTEKSKRFRKKLIERWACEIADFFIKNKVGTVQMENLESMKRKEDSYFNIRLRGFWPYAEMQNKIEFKLKQYGIKIRKVAPNNTSKTCSKCGHLNNYFDFEYRRKSKFPHFKCEKCNFKENADYNAALNISNPKLRSTKEEP

SEQ ID NO: 596 - protein, 726 aa, synthetic construct
SEVEFSHEYWMRHALTLAKRARDEREVPVGAILVLNNRVIGEGWNRAIGLHDPTAHAEIMALRQGGLVMQNYRLIDATLYVTFEPCVMCAGAMIHSRIGRVVFGVRNNKHGAAGSLVNVLNYPGMNHRVEITEGILADECAALLCDFYRMPRQVFNARKKAQSSINPGGSSSGSSGSETPGTSESATPESSGGSSGSSAKNTITKTLKLRIVRPYNSAEVEKIVADEKNNREKIALEKNKDKVKEACSKHLKVAAYCTTQVERNACLFCKARRLDDKFYQKLRGQFPDAVFWQEIGEIFRQLQKQAAEIYNQSLIELYYEIFIKGKGIANASSVEHYLSDVCYTRAAELFKNAAIASGLRNKVKSNFRLKELRSMKSGLPTTKSDNFPIPLVRQKGGQYTGFEISNHNSDFIIKIPFGRWQAKKEIDKYRPWEKFDFEQVRKSPKPISLLLSTQRRKRNRGWSKDESTEAEIKKVMNGDYQTSYIEVKRGSKVGEKSTWMLNLSIDVPKIDKGVDPSIIGGIDVGVKSPLVCAINNAFGRYSISDNDLYRFNKKMFARRRILLKKSKHKRAGHGAKNKLKPITILTEKSGRFRKKLIERWACEIADFFIKNKVGTVQMENLESMKRKEDSYFNIRLRGFWPYAEMQNKIEFKLKQYGIVVRKVAPNNTSKTCSQCGHLNNYFNFEYRKKNKFPYFKCEKCNFKENADYNAALNISNPQLKSTKGEP

SEQ ID NO: 597 - protein, 726 aa, synthetic construct
SEVEFSHEYWMRHALTLAKRARDEREVPVGAVLVLNNRVIGEGWNRAIGLHDPTAHAEIMALHQGGLVMQNYRLIDATLYVTFEPCVMCAGAMIHSRIGRVVFGARNSKRGAAGSLMNVLSYPGMNHRVEITEGILADECAALLRDFYRMPRRVFNAQKKAQSSINSGGSSGGSGGSETPGASESATPKSSVGSSAGSTKSTITKTLKLRIVRPYNSAEVEKIVADEKNNREKIALEKNKDKVKEACSKHLKVAAYCTTQVERSACLFCKARKLDDKFYQKLRGQFPDAVFWQEIGEIFRQLQKQAAEIYNQSLIELYYEIFIKGKGFANASSVEHYLSDVCYTRAAELFKNAAIASGLRGKVKSNFRLKELKNMKSGLPTTKSDNFPIPLVKQKGGQYTGFEISSHNDDFIIKIPFGRWQVKKEVDKYRPWEKFDFEQVRKSPKPISLLLSTQRRKRSKGWSKDEGTEAEIRKVMNGDYQTSYIEVKRGSKTGEKSAWMLNLSIDVPKIDKGVDPSIIGGIDVGVKSPLVCAINNAFSRYSISDNDLFRFNKKMFARRRILLKKNRHKRAGHGAKNKLRPISILTGKSERFRKKLIERWACEIADFFIKNKVGTVQMENLESMKRKEDSYFNIRLRGFWPYAEMQNKIEFKLKQYGIKIRKVAPNNTSKTCSKCGHLNNYFSFEYRKKNKFPHFKCEKCNFKEDADYNAALNISNPKLKSTKEEP

SEQ ID NO: 598 - protein, 726 aa, synthetic construct
SEVEFSHEYWMRHALTLAKRARDEREVPVGAVLVLNNRVIGEGWNRTTGLHDPTAHAEIMALRQGGLVMRNYRLTDATLYVTFEPCVMCAGAMIHSRIGRVVFGVRNSKRGAAGSLMNVLNYPGMNHRVEITEGILADECAALLCDYYRMPRQVFNARKKAQSSINSGGSSDGGSGSETPGTCEGVTPESSGGSSGGSAKNTITKTLKLRIVRPYNSAEVEKIVADEKNNREKIALEKNKDKVKEACSKHLKVAAYCTTQVERNACLFCKARRLDDKFYQKLRGQFPDAVFWQEIGEIFRQLQKQAAEVYNQSLVELYYEILIKGKGIANASSVEHYLSDVCYTRAAELFKNAAIASGLRNKIKSNFRLKELRNMKSGLPTTKSDNFPIPLVRQKGGQYTGFEISNHDGDFIIKIPFGRWQVKKEIDKYRPWEKFDFEQVRKSPKPISLLLSTQRRKRNKGWGKDEGTEAEIKKVMNGDYQTSYIEVKRGGKIGEKSAWMLNLSIDVPKIDKGVDPSIIGGIDVGVKSPLVCAINNAFSRYSISDNDLFRFNKKMFARRRILLKKSKHKRAGHGARNKLKPITILTEKSGRFRKKLIERWACEIADFFIKNKVGTVQMENLESMKRKEDSYFNIRLRGFWPYAEMQNKIEFKLKQYGIVIRKVAPNNTSKTCSKCGHLNNYFNFEYRKKNKFPHFKCEKCNFKENADYNAALNISNPKLKSTKEEP

SEQ ID NO: 599 - protein, 726 aa, synthetic construct
SEVEFSHEYWMRHALTLAKRARDEREVPVGAILVLNNRVIGEGWNRAIGLHDPTAHAEITALRQGGLVMQNYRLIDATLYVTFEPCVMCAGAMIHSRIGRVVFGVRNNKHGAAGSLVNVLDYPGMNHRVEITEGILADECAALLCDFYRMPRQVFNARKKAQSSTNPGGSSGGSSGSETPGTSESATPESSGGNSGGSAKNTITKTLKLRIVRPYNSAEVEKIVADEKNNREKIALEKNRDKVKEACSKHLKVASYCTTQVERNACPFCKARKLDDKFYQKLRGQFPDAVFWQELGEILRQLQKQAAEIYNQSLIELYYEIFIKGKGFANASSVEHYLSDVCYTRAAELFKNAAIASGLRGKVKSNFRLKELKNMKSGLPTTKSDNFPIPLVKQKGGQYTGFEISSHNDDLIVKIPFGRWQVKKEIDRYRPWEKFDFEQVRKSPKPISLLLSTQRRKRNKGWSKDEGTEAEIRKVMNGDYQTSYIEVKRGSKIGEKSAWMLSLSIDVPKIDKGVDPSIVGGIDVGVKSPLVCAINNALGRFSISDNDLFHFNKKMFARRRILLRKNRHKRAGHGAKNKLKPISILTEKSKRFRKKLIERWACEIADFFIKNKVGTVQMENLESMKRKEDSYFNIRLRGFWPYAEMQNKIEFKLKQYGIEIRKVAPNNTSKTCSKCGHLNSYFNFEYRKKNKFPHFKCEKCNFKENADYNAALNISDPKLRSTKEEP

SEQ ID NO: 600 - protein, 726 aa, synthetic construct
SEVEFSHEYWMRHALSLAKRARDEREVPVGAVLVLNNRIIGEGWNRAIGLHDPTAHAEIMALRQGGLVMQNYRLTDATLYVTFEPCVMCAGAMVHSRIGRVVFGVRNSKRGAAGSLMNVLNYPGVNHCVEITEGILVDECAALLCDFYRMPRQVLNAQKKAQSSISSGGSSGGCSGSEMPGASESVTPKSSGGSSGGSAKNTITKTLKLRIVRPYNSAEVEKIVADEKNNREKIALEKNKGKVEEACSKHLKVATYCTTQVERNACLFCRARKLDDKFYQKLRGQFPDAVFWQEIGEIFRQLQKQAAEIYNQSLIELYYEIFIKGKGFANASSVEHYLSDVCYTRAAELFKNAAIASGLRGKVKSNFRLKELKNMRSGLPTTKSDNFPIPLVRQKGGQYTGFEISSHNDDFIIKIPFGRWQVKEEIDKYRPWEKFDFEQVRKNPKPISLLLSIQRRKRNKGWSRDEGTEAEIRKVMNGDYQTSYIEVKRGSKIGEKSAWMLNLSIDVPKIDKGVDPSIIGGIDVGVKSPLICAINNAFSRYGICDNDLFRFNKKVFARRRILLKKNRHKRAGHGTKNKLKPITILTEKSGRFRKKLIERWACEIANFFIKNKVGTVQMENLESMKRKEDSYFNIRLRGFWPYAEMQNKIEFKLRQYGIKIRKVAPNNTSKTCSKCGHLNNYFSFEYRKKNKFPHFKCEKCNFKEDADYNAALNISNPKLKSTKEEP

SEQ ID NO: 601 - protein, 726 aa, synthetic construct
SEVEFSHEYWMRHALSLAKRARDEREVPVGAVLVLNNRIIGEGWNRAIGLHDPTAHAEIMALRQGGLVMQNYRLTDATLYVTFEPCVMCAGAMIHSRIGRVVFGVRNSKRGAAGSLMNVLSYPGMNHRVEITEGILVDECAALLCDFYRMPRQVLNAQKKAQSSISSGGPSGGSSGSETLGASESVTPKSSGGSSAGSTKNTITKTLKLRIVRPYNSAEVEKIVADEKNSREKIALEKNKDKVKEACSKHLKVAAYCTTQVERNACLFCKARRLDDKFYQKLRGRFPDAVFWQEIGEIFRQLQKQAAEIYNQSLIELYYEIFIKGRGFANASSVEHYLSDVCYTRAAGLFKNAAIASGLRGKVKSNFRLKELKNMKSGLPTTKSDNFPIPLVKQKGGQYAGFEISSHNDDFIIKIPFGRWQVKKEIDKYRPWEKFDFEQVRKSPKPISLLLSTQRRKRNKGWSKDEGTEAEIRKVMSGDYQTSYIEVKRGSKTGEKSAWMLNLSIDVPKIDKGVDPSIIGGIDVGVKSPLVCAINNAFSRYSISDNDLFRFNKKMFARRRILLKKNRHKRAGHGAKNKLRPISILTGKGERFRKKLIERWACEIADFFIKNKVGTVQMENLESMKRKEDSYFNIRLRGFWPYAEMQNKIEFKLKQYGIEIRKVAPNNTSKTCSKCGHLNNYFNFEYRKKNKFPHFKCEKCNFKENADYNAALNISNPKLKSTKEEP

SEQ ID NO: 602 - protein, 726 aa, synthetic construct
SEVEFSHEYWMRHALTLAKRARDEREVPVGAILVLNNRVIGEGWNRAIGLNDPTAHAEIMALRQGGLVMQNYRLIDATLYVTFEPCVMCAGAMIHSRIGRVVFGVRNSKRGAAGSLMNVLNYPGMNHCVEITEGILVDECAALLCDFYRMPRQVLNAQKKAQSSISSGGSSGGSSCSETPGASESVTPKSSGGGSAGSTKNTITKTLKLRIVRPYNSAEVEKIVADEKNNREKIALEKNKDKVKEACSKHLKVAAYCTTQVERNACLFCKARRLDDKFYRKLRGQFPDAVFWQEIGEIFRQLQKQAAEIYNQSLIELYYEIFIKGKGFANASSVEHYLSDVCYTRAAELFKNAAIASGLRGKVKSNFRLKELKNMKSGLPTTKSDNFPIPLVKQKGGQYTGFEISSHNDDFIIKIPFGRWQVKKEIDKYRPWEKFDFEQVRKSPKPISLLLSTQRRKRNKGWSKDEGTEAEIRKVMNGDYQTSYIEVKRGCKVGEKSAWMLSLSIDVPKIDKGVDPSIIGGIDVGVKSPLVCAINNAFSRYSISDNDLFHFNKKVFARRRILLKKNRHRRAGHGAKNKLKPITILTEKSKRFRKKLIERWACEIADFFIKNKVGTVQMENLESMKRKEDSYFNIRLRGFWPYAEMQNKIEFKLKQYGIKIRKVAPNNTSKTCSKCGHLNNYFGFEYRRKNKFPHFKCEKCNFKEDADYNAALNISNPKLKSTKEEP

SEQ ID NO: 603 - protein, 726 aa, synthetic construct
SGVEFSHEYWMRHALTLAKRARDEREVPVGAILVLNNRVIGEGWNRAIGLHDPTAHAEIMALRQGGLVMQNYRLIDATLYVTFEPCVMCAGAMVHSRIGRVVFGVRNSKRGAAGSLMNVLNYPGMGHRVEITEGILADECAALLCDFYRMPRQVLSAQKKAQSSISSGGSSGGSSGSETPGASGSVIPKSSGGSSAGSTKDTITKTLKLRIVRPYNSAEVEKVVADEKNNREKIALEKNEGKVKEACSKHLKVATYCTTQVERNACLFCKARKLDDKFYQKLRGQFPDAVFWQELGEIFRQLQKQAAEIYNQSLIELYYEIFIKGKGFANASSVEHYLSDVCYTRAAELFKNAAIASGLRGKVKGNFRLKELKNMKSGLPTTKSDNFPIPLVKQKGGQYTGFEISSHNDDFIIKIPFGRWQAKKEIDKYRPWEKFDFEQVRKSPKPISLLLSTQRRKRNKGWSKDEGTEAEIRKVMNGDYQTSYIEVKRGSKIGEKSTWMLNLSIDVPKIDKGVDPSIIGGIDVGVKSPLICAINNAFSRYGISDNDLFRFNKKVFARRRILLKKNRHKRAGHGTKNKLKPITILTEKSGRFRKKLIERWACEIANFFIKNKVGTVQMENLESMKRKEDSYFNIRLRGFWPYAEMQNKIEFKLKQYGIVVRKVAPNNTSKTCSKCGHLNNYFNFEYRKKNKFPHFKCEKCNFKEDADYNAALNISNPKLKSTKEEP

SEQ ID NO: 604 - protein, 726 aa, synthetic construct
SEVEFSHEYWMRHALTLAKRARDEREVPVGAVLVLNNRVIGEGWNRAIGLHDPTAHAEIMALRQGGLVLQNYRLVDATLYVTFEPCVLCAGAMVHSRIGRVVFGARNSKRGAAGSLMNILNYPGMNHRVEITEGILADECAALLSDFYRMPRQVFNAQKKAQSSINSGGSSGGSSGSETPSTSESATPESSGGSSGGSAKNTITKTLQLRIVRPYNSAEVEKIVTDEKNNREKIALEKNKDKVKEACNKHLKVAAYCTTQVERNACPFCRARKLDDKFYQKLRGQFPDAVFWQELGEIFRQLQKQAAEIYNQSLVELYYEIFIKGKGITNASRVEHYLSDVCYTRAAELFKNAAIASGLRSKVRSNFRLKELKNMKSGLPTTKSDNFPIPLVKQKGGQHTGFEISSHNSDFIIKIPFGRWQVKEEIDKYRPWEKFDFEQVRKSPKPISLLLSTQRRKKNKGWSKDEGTEAEIRRVMNGDYQTSYIEVKRGSKIGEKSAWVLNLSIDVPKIDKGVDPSIIGGIDVGVKSPLVCAINNTFSRYSISDNDLFHFNKKVFARRRILLKKNRHRRAGHGAKNKLKPITILTEKSKRFRKKLIERWACEIADFFIKNKVGTVQMENLESMKRREDSYFNIRLRGFWPYAEMQNKIEFKLKQYGIVVRKVAPNNTSKTCSKCGHLNNYFNFEYRKKNKFPHFKCEKCNFKEGADYNAALNISNPKLKSTRGEP

SEQ ID NO: 605 - protein, 726 aa, synthetic construct
SEVEFSHEYWMRHALTLAKRARDEREVPVGAVLVLNNRVIGEGWNRAIGLHDPTAHAEIMALRQGGLVMQNYRLVDATLYVTFEPCVLCAGAMVHSRIGRVVFGVRNSKRGAAGSLMNVLNYPGMNHRVEITEGILADECAALLCDFYRMPRQVFNAQKKVRSNINSGGSSGGSSASETPGTSESATPESSDGSSGGSAKNTITKTLKLRIVRPYNSAEVEKIVADEKNNREKIALEKNKDKVKEACSKHLKVASYCTTQVERNACPFCKARKLDDKFYQKLRGQFPDAVFWQELGEILRQLQKQAAEIYNQSLIELYYEIFIKGKGFANASSVEHYLSDVCYTRAAELFKNAAIASGLRGKVKSNFRLKEQKNMKSGLPTTKSDNFPIPLVKQKGGQYTGFEISNHNSDFIIKIPFGRWQVKKEINKYRPWEKFDFEQVRKSPKPISLLLSTQRRKRNKGWSKDEGTEAEIRKVMNGDYQTSYIEVKRGSRIGEKSAWMLNLSIDVPKIDKGVDPSIIGGIDVGVKSPLVCAINNAFSRYSISDNDLFRFNKKMFARRRILLGKNRHKRAGHGVKNKLKPITILTEKSGRFRKKLIERWACEIADFFVKNKVGTVQMENLESMKRKEDSYFNIRLRGFWPYAEMQNKIEFKLKQYGIKVRKVAPNNTSKTCSKCGHLNNYFSFEYRKKNKFPHFKCEKCNFKGNADYNAALNISNPKLKSTKEEP

SEQ ID NO: 606 - protein, 726 aa, synthetic construct
SEVEFSHEYWMRHALTLAKRARDEREVPVGAILVLNNRVIGEGWNRAISLHDPTAHAEIMALRQGGLVMQNYRLIDATLYVTFEPCVMCAGAMIHSRIGRVVFGVRNNKHGAAGSLVNVLNYPGMNHRVEITEGILADECAALLCDFYRMPRQVFNARKKAQSSINPGGSSGGSSGSETPGTSESATPESSGGSSGSSAKNTITKTLKLRIVRPYNSAEVEKIVADEKNNREKIALEKNKDKVKEACSKHLKVAAYCTTQVGRNACLFCKARRLDDKFYQKLRGQFPDAVFWQEIGEIFRQLQKQAAEIYNQSLVELYYEIFIKGKGIANASSVEHYLSDVCYTRAAELFKNAAIASGLRNKVKSNFRLKELRSMKSGLPTTKSDNFPIPLVKQKGGQYTGFEISSHNDDFIIKIPFGRWQVKKEIDKYRPWEKFDFEQVRKSPKPISLLLSTQRRKRNKGWSKDEGTEAEIRKVMNGDYQTSYIEVKRGSKIGEKSAWMLSLSIDVPKIDKGVDPSIIGGIDVGVKSPLVCAINNAFCRYSISDNDLFHFNKKMFARRRILLKKSRHKRAGHGAKNKLKPVSILTEKSKRFRKKLIERWACEIADFFIKNKVGTVQMENLESMKRKEDSYFNIRLRGFWPYAEMQNKIEFKLKQYGIEIRKVAPNNTSKTCSKCGHLNNYFNFEYRKKNKFPHFKCEKCNFKENADYNAALNISNPKLKSTKEEP

SEQ ID NO: 607 - protein, 726 aa, synthetic construct
SEVEFSHEYWMRHALTLAKRARDEREVPVGAVLVLNNRVIGEGWNRTTGLHDPTAHAEIMALRQGGLVMRNYRLTDATLYVTFEPCVMCAGAMIHSRIGRVVFGVRNSKRGAAGSLMNVLNYPGMNHCVEITEGILMDECAALLCDFYRMPRQVLNAQKKAQSSISPDGSSGGSSSSETPGTSESATPESSGGNSGGSAKNTITKTLKLRIVRPYNSAEVEKIVADEKNNREKIALEKNRDKVKEACSKHLKVAAYCTTQVERNACLFCKARKLDDKFYQKLRGQFPDAVFWQELGEILRQLQKQAAEIYNQSLIELYYEIFIKGRGFANASSVEHYLSDVCYTRAAELFKNAAIASGLRGKVKGNFRLKELKNMKSGLPTTKSDNFPIPLVKQKGGQYTGFEISNHNSDFIIKIPFGRWQVKKEINKYRPWEKFDFEQVRKSPRPISLLLSTQRRKRNKGWSKDEGTEAEIRKVMNGDYQTSYIEVKRGSKIGEKSAWMLNLSIDVPKIDKGVDPSIIGGIDVGVKSPLVCAIDNAFSRYSISDNDLFHFNKKMFARRRILLRKNRHKRAGHGAKNKLKPITMMTEKSKRFRKKLIERWACEIADFFIKNKVGTVQMENLESMKRKEDSYFNIRLRGFWPYAEMQDKIEFKLKQYGIVVRKVAPNNTSKTCSKCGHLNNYFNFEYRKKNKFPHFKCEKCNFKEDADYNAALNISNPKLKSTKGEP

SEQ ID NO: 608 - protein, 726 aa, synthetic construct
SEVEFSHEYWMRHALTLAKRARGEREVPVGAVLVLNNRVIGEGWNRAIGLHDPTAHAEIMALRQGGLVMQNYRLTDATLYVTFEPCVMCAGAMIHSRIGRVVFGVRNNKHGAAGSLVNVLNYPGMNHRVEITEGILADECAALLCDFYRMPRQVFNARKKARSSINPGGSSGGSSSSETPGASESVTPKSSVGSSAGSTKNTITKTLKLRIVRPYNSAEVEKVVADEKDNREKIALERNKDKVKEACSKHLKVAAYCTTQVERNACLFCKARKLDDKFYQKLRGQFPDAVFWQEIGEIFRQLQKQAAEIYNQSLIELYYEIFIKGKGIANASSVGHYLSDVCYTRAAELFKNAAIASGLRGKIKSNFRLKELKNMKSGLPTTKSDNFPIPLVKQKGGQYTGFEISNHNSDFIIKIPFGRWQVKKEIDKYRPWEKFDFEQVRKSPKPISLLLSTQRRKRNKGWSKDEGTEAEIKRVMNGDYQISYIEVKRGSKIGEKSAWMLSLSVDVPKIDKGVDPSIIGGIDVGVKSPLVCAINNALSRYSISDNDLFHFNKKMFARRRILLRKNRHKRAGHGARNKLKPITVLTEKSERFRKKLIERWACEIANFFIKNKVGTVQMENLESMKRREDSYFNIRLRGFWPYAEMQSKIEFKLKQYGIKIRKVAPNNTSKTCSKCGHLNNYFNFEFRKKNKFPHFKCEKCNFKEDADYNAALNISNPKLKSTKEEP

SEQ ID NO: 609 - protein, 726 aa, synthetic construct
SEVEFSHEYWMRHALTLAKRARDEREVPVGAILVLNNRVIGEGWNRAIGLHDPTAHAEIMALRQGGLVMQNYRLIDATLYVTFEPCVMCAGAMIHSRIGRVVFGVRNSKHGAAGSLVNVLNYPGMNHRVEITEGILADECAALLCDFYRMPRQVFNARKKAQSSINPSGSSGGSSGSVTPGTSESATPESSGGGFGGSAKNTITKTLQLRIVRPYNSAEVEKIVADEKNNREKIALEKYKDKVKEACSKHLKVAAYCTTQVERNACLFCKARKLDDKFYQKLRGQFPDAVFWQEIGEIFRQLQRQAAEIYNQSLIELYYEIFIKGKGFANASSVEHYLSDVCYTRAAELFKNAAIASGLRGKVKSNFRLKELRNMKSGLPTTKSDNFPIPLVKQKGGQYTGFEISSHNDDFIIKIPFGRWQVKKEIDKYRPWEKFDFEQVRKSPKPISLLLSTQRRKRNKGWSKDEGTEAEIRKVMSGDYQTSYIEVKRGSKTGEKSAWMLNLSIDVPKIDKGVDPSIIGGIDVGVKSPLVCAINNALSRYSISDNDLFHFNKKMFARRRILLKKNRRKRAGHGAKNKLKPISILTEKSERFRKKLIERWACEIADFFIKNKVGTVQMENLESMKRREDSYFNIRLRGFWPYAKMLNKIEFKLKQYGIKIRKVAPNNTSKTCSKCGHLNNYFNFEYRKKNKFPHFKCEKCNLKENADYNAALNISNPKLKSTKGEP

SEQ ID NO: 610 - protein, 726 aa, synthetic construct
SEVEFSHEYWMRHALTLARRARDEREVPVGAILVLNNRVIGEGWNRAIGQHDPTAHAEIMALRQGGLVMQNYRLIDATLYVTFEPCVMCAGAMVHSRIGRVVFGVRNSKRGAAGSLMNVLDYPGMGHRVEITEGILADECAALLCDFYRMPRQVFNAQKRAQSSINSGGSSGGSSGSETPGASESVTPKSSGGSSGGSAKNTITKTLKLRIVRPYNSAEVEKIVADEKNNREKIALEKNKGKVKEACSKHLEVAAYCTTQVERNACLFCKARKLDDKFYQKLRGQFPDAVFWQELGGIFRQLQKQAAEIYNQSLIELYYEIFIKGKGITNASRVEHYLSDVCYTRAAELFKNAAIASGLRSKVRSNFRLKELKNMKSGLPTTKSDNFPIPLVKQKGGQYTGFEISSHNSDFIIKIPFGRWQAKKEIDKYRPWEKFDFEQVRKSPKPISLLLSTQRRKRNKGWSKDEGTEAEIRKVMNGDYQTSYIEVKRGSKIGEKSAWMLNLSIDVPKIDKGVDPSIIGGIDVGVKSPLVCAINNAFSRYSISDNDLFHFNKKMFARRRILLKKSRHKRAGHGAKNKLKPISILTEKSKRFRKKLIERWACEIADFFIKNKVGTVQMENLESMKRKEDSYFNIRLRGFWPYAEMQNKIEFKLKQYGIEIRKVAPNNTSKTCSKCGHLNNYFNFEYRKKNKFPHFKCEKCNFKENADYNAALNISNPKLKSTKEEP

SEQ ID NO: 611 - protein, 726 aa, synthetic construct
SEVEFSHEYWMRHALTLAKRARDEREVPVGAVLVLNNRVIGEGWNRAIGLHDPTAHAEIMALRQGGLVLQNYRLADATLYVTFEPCVLCAGAMVHSRIGRVVFGARNSKRGAAGSLMNILNYPGMNHRVEITEGILADECAALLCDFYRMPRQVFNAQKKAQSSINSGGSSGGSSGSETPGTSESATPESSGGSSGGSAKNTITKTLKLRIVRPYNSAEVEKIVADEKNNREKIALEKNKDKVKEACSKHLKVASYCTTQVERNACLFCKARKLDDKFYQKLRGQFPDAVFWQELGGIFRQLQKQAAEIYNQSLIELYYEIFIKGKGITNASRVEHYLSDVCYTRAAELFKNAAIASGLRSKVRSNFRLKELKNMKSGLPTTKSDNFPIPLVKQKGGQYTGFEISSHNDDFIIKIPFGRWQVKEEIDKYRPWEKFDFEQVRKNPKPISLLLSIQRRKRNKGWSRDEGTEAEIRKVMNGDYQTSYIEVKRGSKIGEKSAWMLSLSIDVPKIDKGVDPSIIGGIDVGVKSPLVCAINNAFNRYSISDNNLFHFNKKMFARRRILLKKNRHKRAGHGAKNKLKPISILTEKSERFRKKLIERWACEIADFFIRNKVGTVQMENLEGMKRKEDSYFNIRLRGFWPYAEMQNKIEFKLKQYGIEVRKVAPNNTSKTCSKCGHLNNYFNFEYRRKNKFPHFKCEKCNFKEDADYNAALNISNPKLKSTKEEP

SEQ ID NO: 612 - protein, 726 aa, synthetic construct
SEVEFSHEYWMRRALTLAKRARDEREVPVGAVLVLNNRVIGVGWNRAVGLHDPTAHAEIMALRQGGLVMQNYRLVEATLYVTFEPCIMCAGAMIHSRIGRVVFGVRNSKRGAAGSLMNVLNHPGMNHRVEITEGILADECAALLCDYYRMPRQVFNARKKAQSSINSGGSSDGGSGSETPGTSESATPESSGGSSGGSAKNTITKTLKLRIVRPYNSAEVEKIVADEKNNREKIALEKNKDKVKEACSEHLKVAAYCTTQVERSACLFCKARKLDDKFYQKLRGQFPDAVFWQELGEILRQLQKQAAEIYNQSLIELYYEIFIKGRGFANAGSVEHYLSDVCYTRAAELFKNAAIASGLRGKVKSNFRLKELKNMKSGLPTTKSDNFPIPLVKQKGGQYTGFEISSHNDDFIIKIPFGRWQVKKEIDKYRPWEKFDFEQVRKSPKPISLLLSTQRRKRNKGWSKDEGTEAEIRKVMNGDYQTSYIEVKRGSKTGEKSAWMLNLSIDVPKIDKGVDPSIIGGIDVGVKSPLVCAINNAFSRYSISDNDLFRFNKKMFARRRILLKKNKHKRAGHGAKNKLKPISILTGKSERFRKKLIERWACEIADFFIKNKVGTVQMENLESMKRKEDSYFNIRLRGFWPYAEMQSKIEFKLKQYGIEIRKVAPNNTSKTCSKCGHLNNYFNFEYRKKNKFPHFKCEKCNFKESADYNAALNISNPKLKSTKEEP

SEQ ID NO: 613 - protein, 726 aa, synthetic construct
SEVEFSHEYWMRHALTLAKRARDEREVPVGAVLVLNNRVIGVGWNRAIGLHDPTAHAEIMALRQGGLVMQNYRLTDATLYVTFEPCVMCAGAMVHSRIGRVVFGVRNSKRGAAGSLMNVLNYPGMSHCVEITEGILVDECAALLCDFYRMPRQVLNARKKAQSSISSGGSSGGSGGGETPGASESVTPKSSGGSSAGSTKNTITKTLKLRIVRPYNSAEVEKIVADEKNNREKIALEKNKDKVKEACSKHLKVAAYCTTQVERNACLFCKARKLDDKFYQKLRGQFPDAVFWQELGEIFRQLQKQAAEIYNQSLIELYYEIFIKGKGFANASSVEHYLSDVCYTRAAVLFKNAAIASGLRGKVKSNFRLKELKNMKSGLPTTRSDNFPIPLVKQKGGQYTGFEISSHNDDFIIKIPFGGWQVKKEIDKYRPWEKFDFEQVRKSPKPISLLLSTQRRRRNKGWSKDEGTEAEIRKVMNGDYQTSYIEVKRGSKIGEKSAWMLNLSIDVPKIDRGVDPSIIGGIDVGVKSPLVCAINDAFSRYSISDNELFRFNKKMFARRRILLKKNRHKRAGHGAKNKLKPISILTEKSGRFRKKLIERWACEIADFFIKNKVGTVQMENLEGMKRKEDSYFNIRLRGLWPYAEMQNKIEFKLKQYGIEIRKVAPNNTSKTCSKCGHLNNYFNFEYRKKNKFPHFKCEKCNFKENADYNAALNISNPKLRSTKEEP

SEQ ID NO: 614 - protein, 726 aa, synthetic construct
SEVEFSHEYWMRHALTLAKRARDEREVPVGAILVLNNRVIGVGWNRAIGLHDPTAHAEIMALRQGGLVMQNYRLIDATLYVTFEPCVMCAGAMIHSRIGRVVFGVRNSKHGAAGSLVNVLNYPGMNHRVEITEGILADECAALLCDFYRMPRQVFNARKKAQSSTNSGGPSGGSSGSETPGTSESATPKSSGGSPGGSAKNTITKTLQLRIVRPYNSAEVERIVADEKNNREKIALEKNKDKVREACSKHLKVAAYCTTQVERNACLFCKARKLDDKFYQKLRGQFPDAVFWQELGEILRQLQKQAAEIYNQSLIELYYEIFIKGKGITNASRVEHYLSDVCYTRAAELFKNAAIASGLRSKVRSNFRLKELKNMKSGLPTTKSDNFPIPLVKQKGGQYTGFEISSHNDDFIIKIPFGRWQVKKEIDKYRPWEKFDFEQVRKSPKPISLLLSTQRRKRNKGWSRDEGTEAEIRKVMNGDYQTSYIEVKRGSKTGEKSAWMLNLSIDVPKIDKGVDPSITGGIDVGVKSPLVCAINNAFSRYSISDNDLFRFNKKMFARRRILLKKNRHKRAGHGAKNKLKPISILTGKGERFRKKLIERWACEIADFFIKNKVGTVQMENLESMKRKEDSYFNIRLRGFWPYAEMQNKIEFKLKQYGIEIRKVAPNNTSKTCSKCGHLNNYFNFEYRKKNKFPHFKCEKCNFKENADYNAALNISNPKLKSTKEEP

SEQ ID NO: 615 - protein, 726 aa, synthetic construct
SEVEFSHEYWMRHALTLAKRARDEREVPVGAILVLNNRVIGVGWNRAIGLHDPTAHAEIMALRQGGLVMQNYRLVDATLYVTFEPCVMCAGAMIHSRIGRVVFGVRNSKHGAAGSLVNVLNYPGMNHRVEITEGILADECAALLCDFYRMPRQAFNARKKAQSSINSGGSSGGSSGSETPGTSESATPKSSGGSSGGSAKNTITKALKLRIVRPYNSAEVEKIVADEKDNRERIALEKNKDKVKEACSKHLKVAAYCTTQVERNACLFCKARELDDKFYQKLRGQFPDAVFWQEIGEIFRQLQKQAAEIYNQSLIELYYEIFIKGKGFANASSVEHYLSDVCYTRAAELFKNAAIASGLRGKVKSNFRLKELKNMRSGLPTTKSDNFPIPLVKQKGGQYAGFEISSHNDDFIIKIPFGRWQVKKEIDKYRPWEKFDFEQVRKSPKPISLLLSTRRRKRNKGWSKDEGTEAEIRKVMNGDYQTSYIEVKRGSKIGEKSAWMLNLSIDVPKIDKGVDPGIIGGIDVGVKSPLVCAINNAFGRYSISDNDLFHFNKKMFARRRILLKKNRHKRAGHGAKNKLKPISILTEKSKRFRKKLIERWACEIADFFIKNKVGTVQMENLESMKRKEDSYFNIRLRGFWPYAEMQSKIEFKLKQYGIEIRRVAPNNTSKTCSKCGHLNNYFNFEYRKMNKFPHFKCEKCNFKENADYNAALNISNPKLKSTKEEP

SEQ ID NO: 616 - protein, 726 aa, synthetic construct
SEVEFSHEYWMRHALTLAKRARDEREVPVGAILVLNNRVIGEGWNRAIGLHDPTAHAEIMALRQGGLVTQNYRLIDATLYVTFEPCVMCAGAMIHSRIGRVVFGVRNSKHGAAGSLVNVLNYPGMNHRVEITEGVLADECAALLCDFYRMPRQVFNARKKAQSNINPGGSSGGSSGSETPGTSDSATPGSSGGSSGGSAKNTITKTLKLRIVRPYNSAEVEKIVADEKNNREKTALEKNKDKVKEACSKHLKMASYCTTQVERNACLFCKARKLDDKFYQKLRGQFPDAVFWQELGGIFRQLQKQAAEIYNQSLIELYYEIFIKGRGFANASSVEHYLSDVCYTRAAELFKNAAIASGLRGKVKSNFRLKELKNMKSGLPTTKSDNFPIPLVKQKGGQYTGFEISSHHDDFVIKIPFGRWQVKKEIDKYRPWEKFDFEQVRKSPKPISLLLSTQRRKRNKGWSKDEGTEAEIRKVMNGDYQTSYIEVKRGSKIGEKSAWMLNLSIDVPKIDKGVDPSIIGGIDVGVKSPLVCAINNALSRYSISDNDLFHFNKKMFARRRILLRKNRHKRAGHGAKNKLKPITIMTEKSKRFRKKLIERWACEIADFFIKNKVGTVQMENLESMKRREDSYFNIRLRGFWPYAEMQNKIEFKLKQYGIVVRKVAPNNTSKTCSKCGHLNNYFNFEYRKKNKFPHFKCEKCNFKEDADYNAALNISNPKLKSTKGEP

SEQ ID NO: 617 - protein, 726 aa, synthetic construct
SEVEFSHEYWMRRALTLAKRARDEREVPVGAVLVLNNRVIGEGWNRAIGLHDPTAHAEIMALRQGGLVMQNYRLTDATLYVTFEPCVMCAGAMIHSRIGRVVFGVRNSKRGAAGSLLNVLNYPGMNHCVEITEGILVDECAELLCDFYRMPRQVLNAQKKAQSSISSGGSSGGSSGSETPGASESATPKSSGGSSASSTKNTITKTLKLRIVRPYNSAEVEKIVADEKNNRERIALEKNKDKVKEACSKHLKVAAYCTTQVERNACLFCKARKLDDKFYQKLRGQFPDAVFWQETGEIFRQLQRQAAEIYNQSLIELYYEIFIKGRGFANASSVEHYLSDVCYTRAAELFKNAAIASGLRGKVKGNFRLKELKNMKSGLPTTKSDNFPIPLVKQKGGQYTGFEISSHNDDFIIKIPFGRWQAKKEIDKYRPWEKFDFEQVRKSPKPISLLLSTQRRKRNKGWSKDEGTEAEIRKVMNGDYQTSYIEVKRGSKIGEKSAWMLNLSIDVPKIDKGVDPSIIGGIDVGVKSPLVCAINNAFSRYSISDNDLFHFNKKMFARRRILLKKNRHRRAGHGAKNKLKPISILTEKSKRFRKKLIERWACEIADFFIKNKVGTVQMENLESMKRKEDSYFNIRLRGFWPYAEMQNKIEFKLKQYGIEIRRVAPNNTSRTCSKCGHLNNYFNFEYRRKYKFPHFKCEKCNFKEDADYNAALNISNPKLKSTKEEP

SEQ ID NO: 618 - protein, 726 aa, synthetic construct
SEVEFSHEYWMRHALTLAKRARDEREVPVGAVLVLNNRVIGEGWNRAIGLYDPTAHAEIMALRQGGLVMQNYRLTDATLYVTFEPCVMCAGAMIHSRIGRVVFGVRNSKRGAAGSLMNVLNYPGMNHCVEITEGILVDECAALLCDFYRMPRQVLNAQKKAQPSINSGGSSGGGSGSETPGTSESATPESSGGGSSGSAKNTITKTLQLRIVRPYNSAEVEKVVADEKNNREKIALEKNKDKVKEACSKHLKVASYCTTQVERNACPFCKARKLDDKFYQKLRGQFPDAVFWQELGEILRQLQKQAAEIYNQSLIELYYEIFIKGRGFANASSVEHYLSDVCYTRAAELFKNAAIASGLRGKVKSNFRLKELKNMKSGLPTTKSDNFPIPLVKQKGGQYTGFEISSHNDDFIIKIPFGRWQVKEEIDKYRPWEKFDFEQVRKNPKPISLLLSTQRRKRNKGWSKDEGTEAEIRKVMNGDYQTSFIEVKRGSKIGEKSAWMLSLSIDVPKIDKGVNPSIIGGIDVGVRSPLVCAINNAFSRYSISDNDLFHFNKKMFARRRILLKKNRHKRAGHGAKNKLKPISILTEKSKRFRKKLIERWACEIADFFIKNKVGTVQMENLESMKRKEDSYFNIRLRGFWPYAEMQNKIEFKLKQYGIKVRKVAPNNTSKTCSKCGHLNNYFSFEYRKRNKFPHFKCEKCNFKENADYNAALNISNPKLKSTKEKP

SEQ ID NO: 619 - protein, 726 aa, synthetic construct
SEVEFSHEYWMRHALTLAKRARDEREVPVGAILVLNNRVIGEGWNRAIGLHDPTAHAEIMALRQGGLVMQNYRLIDATLYVTFEPCVMCAGAMIHSRIGRVVFGVRNNKHGAAGSLVNVLNYPGMNHRVEITEGILVDECAALLCDFYRMPRQVFNARKKAQSSINSGGSSGGSSGSETPGTSESPTPESSGGSPGGSAKNTITKTLKLRIVRPYNSAEVEKIVADEKNNREKVALEKNKDKVKEACSEHLKVAAYCTTQVERSACLFCKARKLDDKFYQKLRGQFPDAVFWQEIGEIFRQLQKQAAEIYNQSLIELYYEIFIKGKGFANASSVEHYLSDVCYTRAAELFKNAAIASGLRGKVKSNFRLKELKNMKSGLPTTKSDNFPIPLVKQKGGQYTGFEISSHNDDFIIKIPFGRWQVKKEIDKYRPWEKFDFEQVRKSPKPISLLLSTQRRKRNKGWSKDEGTEAEIRKVMNGDYQTSYIEVKRGSKIGEKSAWMLNLSIDVPKIDKGVDPSVIGGIDVGVKSPLVCAINNALSRYSISDNDLFHFNKKMFARRRILLRKNRHKRAGHGAKNKLKPITILTEKSKRFRKKLIERWACEIADFFIKNKVGTVQMENLESMKRREDSYFNIRLRGFWPYAEMQNKIEFKLKQYGIEIRKVAPNNTSKTCSKCGHLNNYFNFEYRKKNKFPHFKCEKCNFKENADYNAALNISNPKLKSTKEEP

SEQ ID NO: 620 - protein, 726 aa, synthetic construct
SEVEFSHEYWMRHALTLAKRARDEREVPVGAVLVLNNRVIGEGWNRAIGLHDPTAHAEIMALRQGGLAMQNYRLVDATLYVTFEPCVLCAGAMVHSRIGRVVFGARNSKRGAAGSLMNILNYPGMNHRVEITEGILADECAALLCDFYRMPRQVFNAQKKAQSSINSGGSSGGSSGSETPSTSESATPESSGGSSGGSARNTITKTLQLRIVRPYNSAEVEKIVTDEKNNREKIALEKNKDKVKEACSKHLKMASYCTTQVERNACLFCKARKLDDKFYQKLRGQFPDAVFWQELGGIFRQLQKQAAEIYNQSLIELYYEIFIKGKGFTNASRVEHYLSDVCYTRAAELFKNAAIASGLRSKVRSNFRLKELKNMKSGLPTTKSDNFPIPLVKQKGGQYTGFEISSHNSDFIIKIPFGRWQVKEEIDKYRPWEKFDFEQVRKSPKPISLLLSTQRRKRNKGWSKDEGTEAEIRKVMNGDYQTSYIEVKRGSKIGEKSAWMLNLSIDVPKIDKGVDPSIIGGIDVGVKSPLVCAINNAFSRYSIGDNDLFHYNKKMFARRRILLKKNRHKRAGHGAKNKLKPISILTEKSKRFRKKLIERWACEIADFFIRNKVGTVQIENLESMKRKEDSYFNIRLRGFWPYAEMQNKIEFKLKQYGIEIRKVAPNNTSKTCSKCGHLNSYFNFEYRKKNKFPHFKCEKCNFKENADYNAALNISNPKLKSTKEEP

SEQ ID NO: 621 - protein, 726 aa, synthetic construct
SEVEFSHEYWMRHALTLAKRARDEREVPVGAVLVLDNRVIGVGWNRAIGLHDPTAHAEIMALRQGGLVMQNYRLTDATLYVTFEPCVMCAGAMVHSRIGRVVFGVRNSKRGAAGSLMNVLNYPGMSHCVEITEGILVDECAALLCDFYRMPRQVLNAQKKAQSSISSGGSSGGSGGGETPGTSESATPESSGGGSSGSAKNTITKTLQLRIVRPYNSVEVEKIVADEKNNREKIALEKNKDKVREACSKHLKVASYCTTQVERNACPFCKARKLDDKFYQKLRGQFPDAVFWQELGEILRQLQKQAAEIYNQSLVELYYEIFIKGKGFANASSVEHYLSDVCYTRAAELFKNAAIASGLRGKVKSNFRLKELKNMKSGLPTTKSDNFPIPLVKQKGGQYTGFEISSHNDDFVIKIPFGRWQVKEEIDKYRPWEKFDFEQVRKNPKPISLLLSTQRRKGNKGWSKDEGTEAEIRKVMNGDYQTSYIEVKRGSKIGEKSAWMLNLSIDVPKIDKGVDPSIIGGIDVGVKSPLVCAINNAFSRYSISDNDLFRFNKKVFARRRILLKKNRHKRAGHGTKNKLKPITILTEKSGRFRKKLIERWACEIANFFVKNKVGTVQMENLESMKRREDSYFNIRLRGFWPYAEMQNKIEFKLRQYGIKIRKVAPNNTSKTCSKCGHLNNYFSFEYRKKNKFPHFKCEKCNFKEDADYNAALNISNPKLKGTKEEL

SEQ ID NO: 622 - protein, 726 aa, synthetic construct
SEVEFSHEYWMRHALTLAKRARDEREVPVGAVLVLNNRVIGEGWNRAIGLHDPTAHAEIMALRQGGLVMQNYRLVDATLYVTFEPCVLCAGAMVHSRIGRVVFGVRNSKRGAAGSLMNVLNYPGMNHRVEITEGILADECAALLCDFYRMPRQVFNARKKARSNINSGGSSGGSSGSETLGTREGATPESSGGSSGGSAKNTITKTLKLRIVRPYNSAEVEKIVADEKNSREKIALERNKDKVKEACSKHLKVASYCTTQVERNACPFCKARKLDDKFYQKLRGQFPDAVFWQELGEILRQLQKQAAEIYNQSLIELYYEIFIKGRGFANASSVEHYLSDVCYTRAAELFKNAAIASGLRGKVKSNFRLKELRNMKSGLPTTKSDNFPIPLVKQKGGQYTGFEISNCDSDFVIKIPFGRWQAKKEIDKYRPWERFDFEQVRKSPKPISLLLSTQRRKRNKGWSKDEGTEAEIKKVMNGDYQISYIEVKRGSKIGEKSAWMLNLSIDVPKIDKGVDPSIVGGIDVGVKSPLVCAINNAFSRYSISDNDLFHFNKKVFARRRILLKKNRHRRAGHGAKNKLKPITILTEKSKRFRKKLIERWACEIADFFIKNKVGTVQMENLESMKRREDSYFNIRLRGFWPYAEMQNKIEFKLKQYGIEIRKVAPNNTSRTCSKCGHLNNYFNFEYRKKNKFPHFKCEKCNFKEDADYNAALNISNPKLKSTKEES

SEQ ID NO: 623 - protein, 726 aa, synthetic construct
SEVEFSHEYWMRHALTLAKRARDEREVPVGAVLVLNNRVIGEGWNRAIGLHDPTAHAEIMALRQGGLAMQNYRLVDATLYVTFEPCVMCAGAMIHSRIGRVVFGVRNSKRGAAGSLMNVLNYPGMNHRVEITEGILADECAAPLCDFYRMPRQVFNAQKKAQSSINSGGSSDGGSGSETPGTSESATPESSGGSSGGSAKNTITKTLKLRIVRPYNSAEVEKIVADEKNNREKIALEKNKDKVKEACSEHLKVAAYCTTQVERSACLFCKARKLDDKFYQKLRGQFPDAVFWQEIGEIFRQLQKQAAEIYNQSLIELYYEIFIKGKGSANASSVEHYLSDVCYTRAAEQFKNAAIASGLRNKIKSNFRLKELRNMKSGLPTTKSDNFPIPLVRQKGGQYTGFEISNHNGDFIIKIPFGRWQVKKEIDKYRPWEKFDFEQVRKSPKPISLLLSTQRRKRNKGWSKDEGTEAEIRKVMSGDYQTSYIEVKRGSKTGEKSAWMLNLSIDVPKIDKGVDPSIIGGIDVGVKSPLVCAINNAFSRYSISDNDLFRFNKKMFARRRILLKKNRHKRAGHGAKNKLKPITILTKKSERFRKKLIERWACEIADFFIKNKVGTVQMENLESMKRKEDSYFNIRLRGFWPYAEMQNKIEFKLKQYGIEIRKVAPNNTSKTCSKCGHLNHYFNFEYRRKNKFPHFKCEKCNFRENADYNAALNISNPKLKSTKGEP

SEQ ID NO: 624 - protein, 726 aa, synthetic construct
SEDEFSHEYWMRHALTLAKRARDGREVPVGAVLVLNNRVIGEGWNRAIGLHDPTAHAEIMALRQGGLVMQNYRLIDATLYVTFEPCVMCAGAMVHSRIGRVVFGVRNSKRGAAGSLMNVLNYPGMGHRVEITEGILADECAALICDYYRMPRQVFSARKKAQSSINSGGSSDGGSGSETPGTSESPTPESPGGSSGGSAKNTITKTLKLRIVRPYNSAEVEKIVADEKNNREKIALEKNKDKVKEACSKHLKVASYCTTQVERNACPFCKARKLDDKFYQKLRGQFPDAVFWQELGEILRQLQKQAAEIYNQSLIELYYEIFIKGKGFANASSVEHYLSDVCYTRAAELFKNAAIASGLRGKVKSNFRLKELKNMKSGLPTTKSDNFPIPLVKQKGGQYTGFEISSHNDDFIIKIPFGRWQVKEEIDKYRPWEKFDFEQVRKNPKPISLLLSTQRRKRNKGWSKDEGTEAEIRKVMNGDYQTSYIEVKRGSKIGEKSAWMLNLSIDVPKIDKGVDPSIIGGIDVGVKSPLVCAINNAFSRYSISDNDLFRFNKKVFARRRILLKKNRHKRAGHGTKNKLKPITILTEKSGRFRKKLIERWACEIANFFIKNKVGTVQMENLESMKRKEDSYFNIRLRGFWPYAEMQNKIEFKLKQYGIKIRKVAPNNTSKTCSKCGHLSNYFSFEYRKKNKFPHFKCEKCNFKEDADYNAALNISNPKLKSTKEEP

SEQ ID NO: 625 - protein, 726 aa, synthetic construct
SEVEFSHEYWMRHALTLAKRARDEREVPVGAVLVLNNRVIGVGWNRAIGLHDPTAHAEIMALRQGGLVLQNYRLVDATLYVTFEPCVLCAGAMVHSRIGRVVFGARNSKRGAAGSLMNILNYPGMNHRVEITEGILADECAALLCDFYRMPRQVFNAQKKAQSSINSGGSSGGSSGSETPSTSESATPESSGGSSGGSAKNTITKTLQLRIVRPYNSAEVEKIVTDEKNNREKIALEKNKDKVKEACSKHLKMASYCTTQVERNACLFCKARKLDDKFYQKLRGQFPDAVFWQELGGIFRQLQKQAAEIYNQSLIELYYEIFIKGKGITNASRVEHYLSDVCYTRAAELFKNAAIASGLRGKVKSNFRLKELKNMKSGLPTTKSDNFPIPLVKQKGGQYTGFEISSHNDDFIIKIPFGRWQVKKEIDKYRPWEKFDFEQVRKSPKPISLLLSTQRRKRNKGWSKDEGTEAEIRKVMNGDYQTSYIEVKRGSKTGEKSAWMLNLSIDVPKIDKGVDPSIIGGIDVGVKSPLVCAINNAFSRYSISDNDLFRFNKKMFARRRILLKKNRHKRAGHGAKNKLKPISILTGKSERFRKKLIERWACEIADFFIKNKVGTVQMENLESMKRKEDSYFNIRLRGFWPYAEMQNKIEFKLKQYGIEIRKVAPNNTSKTCSKCGHLNNYFSFEHRKKNKFPHFKCEKCNFKENADYNAALNISNPKLKSTKEEP

SEQ ID NO: 626 - protein, 726 aa, synthetic construct
SEDEFSHEYWMRHALTLAKRARDGREVPVGAVLVLNNRVIGEGWNRAIGLHDPTAHAEIMALRQGGLVMQNYRLIDATLYVTFEPCVMCAGAMVHSRIGRVVFGVRNSKRGAAGSLMNVLDYPGMGHRVEITEGILADECAALLCDFYCMPRQVFNAQKRAQSSINPGGSSGGSSGSETPGTSESATLENSGGSSGGSAKNTITKTLKLRIVRPYNSAEVERIVADEKNNREKIALEKNKDKVKEACSKHLKVAAYCTTQVERNACLFCKARRLDDKFYQKLRGQFPDAVFWQELGEIFRQLQKQAAEIYNQSLIELYYEIFIKGRGFANASSVEHYLSDVCYTRAAELFKNAAIASGLRGKVKSNFRLKELKNMKSGLPTTKSDNFPIPLVKQKGGQYTGFEISSHNDDFIIKIPFGRWQVKKEIDKYRPWEKFDFEQVRKSPKPISLLLSTQRRKRNKGWSKDEGTEAEIRKVMNGDYRTSYIEVKRGSKTGEKSAWVLNLSIDVPKIDKGVDPSIIGGIDVGVKSPLVCAINNAFSRYSISDNDLFRFNKKMFARRRILLKKNRHKRAGHGAKNKLKPISILTGKSERFRKKLIERWACEIADFFIKNKVGTVQMENLESMKKKEDSYFNIRLRGFWPYAEMQNKIEFKLKQYGIEIRKVAPNNTSKTCSKCGHLNSYFNFEYRKKNKFPHFKCEKCNFKENADYNAALNISNPKLKSTKEEP

SEQ ID NO: 627 - protein, 726 aa, synthetic construct
SEVEFSHEYWMRHALTLAKRARDEREVPVGAILVLNNRVIGEGWNRAIGLHDPTAHAEIMALRQGGLVMQNYRLIDATLYVTFEPCVMCAGAMIHSRIGRVVFGVRNNKHGAAGSLVNVLDYPGMNHRVEITEGILADECAALLCDFYRMPRQVFNARKKAQSSISPGGSSGGSSGSETPGTSESVTPESSGGSPGGSAKNTITKTLKLRIVRPYNSAEVEKIVADEKNNREKIALEKNKDKVREACSKHLKVAAYCTTQVERNACLFCKARRLDDKFYQKLRSQFPDAVFWQEIGEIFRQLQKQAAEIYNQSLVELYYEILIKGKGIANASSVEHYLSDVCYTRAAELFKNAAIASGLRNKIKSNFRLKELRNMKSGLPTTKSDNFPIPLVKQKGGQYTGFEISSHNDDFIIKIPFGRWQVKKEIDKYRPWEKFDFEQVRKSPKPISLLLSTQRRKRNKGWSKDEGTEAEIRKVMNGDYQTSYIEVKRGSKIGEKSAWMLNLSIDVPKIDKGVDPSIIGGIDVGVKSPLVCAINNAYSRYSIGDNDLFHYNKKMFARRRILLKKNRHKRAGHGAKNKLKPISILTEKSKRFRKKLIERWACEIADFFIKNKVGTVQMENLESMKRREDSYFNIRLRGFWPYAEMQSKIEFKLKQYGIKIRKVAPNNTSKTCSRCGHLNNYFNFEYRRKNKFPHFKCEKCNFKENADYNAALNISNPKLKSTKEEP

SEQ ID NO: 628 - protein, 726 aa, synthetic construct
SEVEFSHEYWMRHALTLARRARDEREVPVGAILVLNNRVIGEGWNRAIGLHDPTAHAEIMALRQGGLVMQNYRLVDATLYVTFEPCVMCAGAMIHSRIGRVVFGVRNNKHGAAGSLMNVLNYPGMNHRVEITEGILADECAALLCDFYRMPRQVFNARKKAQSSISSGGSSGGSSGSETPGASESVTPKSSGGGSAGSTKNTITKTLKLRIVRPYNSAEVEKIVADEKNSREKIALEKNKDKVKEACSKHLKVASYCTTQVERNACLFCKARKLDDKFYQKLRGQFPDAVFWQELGEIFRQLQKQATEIYNQSLIELYYEIFIKGKGFANASSVEHYLSDVCYTRAAELFKNAAIASGLRGKVKSNFRLKELKNMKSGLPTTKSDNFPIPLVKQKGGQYTGFEISSHNSDFIIKIPFGRWQVKEEIDKYRPWEKFDFEQVRKSPKPISLLLSTQRRKRNKGWGKDEGTEAEIRKAMNGDYQTSYIEVKRGSKIGEKSAWMLSLSIDVPKIDKGVDPRTIGGIDVGVKSPLVCAINNVLSRYSISDNDLFHFNKKMFARRRILLKKNGHKRAGHGAKNKLKPITLMTEKSKRFRKKLIERWACEIADFFIKNKVGTVQMENLESMKRKEDSYFNIRLRGFWPYAEMQNKIEFKLKQYGIVVRKVAPNNTSKTCSQCGHLNDYFNFEYRKKNKFPHFKCEKCNFKENADYNAALNISNPKLKSIKEGP

SEQ ID NO: 629 - protein, 726 aa, synthetic construct
SEVEFSHEYWMRHALTLAKRARDEREVPVGAVLVLNNRVIGEGWNRAIGLHDPTAHAEIMALRQGGLVMQNYRLVDATLYVTFEPCVLCAGAMVHSRIGRVVFGVRNSKRGAAGSLMNVLNYPGMNHRVEITEGILADECAALLCDFYRMPRQVFNARKKARSNINSGGSSGGSSGSETLGTREGATPESSGGSSGGSAKNTITKTLKLRIVRPYNSAEVEKIVADEKNNREKIALEKNKDKVKEACSKHLKVAAYCTTQVERNACLFCKARKLDDKFYQKLRGQFPDAVFWQELGEILRQLQKQAAEIYNQSLIELYYEIFIKGRGFANASSVEHYLSDVCYTRAAELFKNAAIASGLRGKVKGNFRLKELKNMKSGLPTTKSDNFPIPLVKQKGGQYTGFEISSHNDDFIIKIPFGRWQVKKEIDKYRPWEKFDFEQVRKSPKPISLLLSTQRRKRNKGWSKDEGTEAEIRKVMNGDYQTSYIEVKRGSKTGEKSAWMLNLSIDVPKIDKGVDPSIIGGIDVGVKSPLVCAINNAFSRYSISDNDLFRFNKKMFARRRILLGKNRHKRAGHGVKNKLKPITILTEKSGRFRKKLIERWACEIADFFVKNKVGTVQMENLESMKRKEDSYFNIRLRGFWPYAEMQDKIEFKLKQYGIEIRKVAPNNTSKTCSKCGHLNNYFNFEYRKKNKFPHFKCERCNFKENADYNAALNISNPKLKSTKEKP

SEQ ID NO: 630 - protein, 726 aa, synthetic construct
SEVEFSHEYWMRHALSLAKRARDEREVPVGAVLVLNNRIIGEGWNRAIGLHDPTAHAEIMALRQGGLVMQNYRLTDATLYVTFEPCVMCAGAMVHSRIGRVVFGVRNSKRGAAGSLMNVLNYPGVNHCVEITEGILVDECAALLCDFYRMPRQVLNAQKKAQSSINPGGPSGGSSGSETPDTSESPTPESSGGSSGGSAKNTITKTLKLRIVRPYNSAEVEKIVADEKNNREKIALEKNKDKVKEACSEHLKVAAYCTTQVERNACLFCKARKLDDKFYQKLRGQFPDAVFWQELGEIFRQLQKQAAEIYNQSLIELYYEIFIKGRGFANASSVEHYLSDVCYTRAAGLFKNAAIASGLRGKVKSNFRLKELKNMKSGLPTTKSDNFPIPLVKQKGGQYTGFEISNHNDDFIIKIPFGRWQAKKEIDRYRPWEKFDFEQVRKNPKPISLLLSTRRRKRNKGWSKDEGTEAEIRRVMNGDYQTSYIEVKRGSKTGEKGAWMLNLSIDVPKIDKGVDPSIIGGIDVGVKSPLVCAVNNAFSRYSISDNDLFRFNKKMFARRRILLGKNRHKRAGHGAKNKLKPISILTEKSKRFRKKLIERWACEIADFFIKNKVGTVQMENLESMKRKEDSYFNIRLRGFWPYAEMQNKIEFKLRQYGIEIRKVAPNNTSKTCSRCGHLNNYFNFEYRRKNKFPHFKCEKCNFKENADYNAALNISNPKLKSTKEEP

SEQ ID NO: 631 - protein, 726 aa, synthetic construct
SEVEFSHEYWMRHALTLAKRARDEREVPVGAILVLNNRVIGEGWNRAIGLHDPTAHAEIMALRQGGLVMQNYRLIDATLYVTFEPCVMCAGAMIHSRIGRVVFGVRNSKHGAAGSLVNVLNYPGMNHRVEITEGILADECAALLCDFYRMPRQVFGARRKTQSSINPGGSSGGSSGSETPGTSESPTPESPGGNSGGSAKNTITKTLKLRIVRPYNSAEVEKIVADEKNNRERIALEKNKDKVKEACSKHLKVAAYCTTQVERNACLFCKARKLDDKFYQKLRGQFPDAVFWQEIGEIFRQLQKQAAEIYNQSLIELYYEILIKGKGFANASSVEHYLSDVCYTRAAELFKNAAIASGLRGKVKSNFRLKELKNMRSGLPTTKSDNFPIPLVKQKGGQYAGFEISSHNDDFIIKIPFGRWQVKKEIDKYRPWEKFDFEQVRKSPKPISLLLSTRRRKRNKGWSKDEGTEAEIRKVMNGDYQTSYIEVKRGSKIGEKSAWMLNLSIDVPKIDKGVDPSIIGGIDVGVKSPLVCAINNAFSRYSISDNDLFRFNKKMFARRRILLKKNRHKRAGHGAKNKLKPISILTEKSKRFRKKLIERWACEIADFFIKNKVGTVQMENLESMKRKEDSYFNIRLRGFWPYAEMQNKIEFKLKQYGIEIRKVAPNNTSKTCSKCGHLNNYFNFEYRKRNKFPHFKCEKCNFKEDADYNAALNISNPKLKGTKEEP

SEQ ID NO: 632 - protein, 726 aa, synthetic construct
SEVEFSHEYWMRHALTLAKRARDEREVPVGAVLVLNNRVIGEGWNRAIGLHDPTAHAEIMALRQGGLVMQNYRLTDATLYVTFEPCVMCAGAMIHSRIGRVVFGVRNSKRGAAGSLMNVLNYPGMNHCVGITEGILVDECAALLCDFYRMPRQVLNAQKKAQSSISSGGSSGGSSGSETPGASESATPKSSGGSPGGSAKNTITKTLKLRIVRPYNSAEVEKIVADEKNNREKIALEKNKDKVKEACSKHLKVAAYCTTQVERNACLFCKARRLDDKFYQKLRGQFPDAVFWQEIGDIFRQLQKQAAEIYNQSLIELYYEIFIKGRGFANASSVEHYLSDVCYTRAAELFKNAAIASGLRGKVKSNFRLKELKSMKSGLPTTKSDNFPIPLVKQKGGQYTGFEISSHNDDFIIKIPFGRWQVKKEINKYRPWEKFDFEQVRKSPKPISLLLSTRRRKRNKGWSKDEGTEAEIRKVMNGDYQTSYIEVKRGSKIGEKSAWMLNLSIDVPKIDKGVDPSIIGGIDVGVKSPLVCAINNAFGRYSISDNDLFHFNKKMFAMRRILLKKNRHKRAGHGAKNKLRPITILTEKSKRFRKKLIERWACEIADFFIKNKVGTVQMENLESMKRKEDSYFNIRLRGFWPYAEMQNKIEFKLKQYGIEIRKVAPNNTSKTCSKCGHLNYYFNFEYRKKNKFPHFKCEKCNFKEDADYNAALNISNPKLKSTKEEP

SEQ ID NO: 633 - protein, 726 aa, synthetic construct
SEVEFSHEYWMRRALTLAKRARDEREVPVGAVLVLNNRVIGVGWNRAVGLHDPTAHAEIMALRQGGLVMQNYRLIEATLYVTFEPCIMCAGAMIHSRIGRVVFGVRNSKRGAAGSLMNVLNYPGMNHRVEITEGILADECAALLCDYYRMPRQVFNAQKRAQSSINSGGSSGSSSGSETPGTSESATPESSGGSSAGSTKDTITKTLKLRIVRPYNSAEVEKIVADEKNNREKIALEKNKDKVKEACSKHLKVAAYCTTQVERNACLFCKARKLDDKFYQKLRGQFPDAVFWQEISEIFRQLQKQAAEIYNQSLIELYYEIFIKGKGFANASSVEHYLSDVCYTRAAELFKNAAIASGLRGKVKSNFRLKELKNMRSGLPTTKSDNFPVPLVKQKGGQYTGFEISNHNSDFIIKIPFGRWQVKEEINKYRPWEKFDFEQVRKSPKPISLLLSTQRRKRNKGWSKDEGTEAEIRKVMNGDYQTSYIEVRRGSKIGERSAWMLNLSIDVPKIDKGVNPSIIGGIDVGVRSPLVCAINNALSRYSISDNDLFHFNKKMFARRRILLRKNRHKRAGHGAKNKLKPITMMTEKSKRFRKKLIERWACEIADFFVKNKVGTVQMENLESMKGKEDSYFNIRLRGFWPYAEMQNKIEFKLKQYGIKIRKVAPNNTSKTCSKCGHLNDYFNFEYRRKNKFPHFKCEKCYFKEDADYNAALNISNPKLKSTKEEP

SEQ ID NO: 634 - protein, 726 aa, synthetic construct
SEVEFSHEYWMRHALTLAKRARDEREVPVGAVLVLNNRVIGEGWNRAIGLHDPTAHAEIMALRQGGLVTQNYRLIDATLYVTFEPCVMCAGAMVHSRIGRVVFGVRNSKRGAAGSLMNVLNYPGMNHCVEITEGILVDECAALLCDFYRMPRQVLNAQKKAQSSISSGGSSGGSNGSETPCASESATPKSSGGSSAGSTKNTITKTLKLRIVRPYNSAEVEKIVTDEKNNREKIALEKNKDKVKEACSKHLKMAAYCTTQVERNACLFCRARKLDDKFYQKLRGQFPDAVFWQELGEILRQLQKQAAEIYNQSLIELYYEIFIKGRGFANASSVEHYLSDVCYTRAAELFKNAAIASGLRGKVKSNFRLKELKNMRSGLPTTKSDNFPIPLVKQKGGQYTGFEISSHNDDFIIKIPFGRWQVKKEIDKYRPWERFDFEQVRKSPKPISLLLSTQRRKRNKGWSKDEGTEAEIRKVMNGNYQTSYIEVRRGSKIGEKSAWMLNLSIDVPKIDKGVDPSVIGGIDVGVKSPLVCAINNAFSRYSISDNDLFHFNKKVFARRRILLKKNRHRRAGHGAKNKLKPITILTEKSKRFRKKLIERWACEIADFFIKNKVGTVQMENLESMKRKEDSYFNIRLRGFWPYAEMQNKIEFKLKQYGIEIRKVAPNNTSKTCSKCGHLNNYFNFEYRKKNKFPPFKCEKCNFKEDADYNAALNISNPKLKGTKEEP

SEQ ID NO: 635 - protein, 726 aa, synthetic construct
SEVEFSHEYWMRYALTLAKRARDEREVPVGAVLVLNDRVIGEGWNRAIGLHDPTAHAEIMALRQGGLVMQNYRLIDATLYVTFEPCVMCAGAMIHSRIGRVVFGVRNNKHGAAGSLVNVLNYPGMNHRVEITEGILADECAALLCDFYRMPRQVFNARKKAQSSINPGGSSGGSSGSETPGTSESATPESSGGSSGSSAKNTITKTLKLRIVRPYNSAEVEKIVADEKNNREKIALEKNKDKVKEACSKHLKVAAYCTTQVERNACLFCKARKLDDKFYQKLRGQFPDAVFWQEIGEIFRQLQKQAAEIYNQSLIELYYEIFIKGKGFANASSVEHYLSDVCYTRAAELFKNAAIASGLRGKVKSNFRLKELKNMKSGLPTTKSDNFPIPLVKQKGGQYAGFEISSHNDDFVIKIPFGRWQVKKEIDKYRPWEKFDFEQVRKSPKPISLLLSTQRRKRNKGWSKDEGTEAEIRKVMNGDYQTSYIEVKRGSKIGEKSAWMLNLSIDVPKIDKGVNPSIIGGIDVGVKSPLVCAINNAFSRYSISDNDLFHFNKKMFARRRILLKKNRHKRAGHGAKNKLKPISILTEKSKRFRKKLIERWACEIADFFIKNKVGTVQMENLESMKRKEDSYFNIRLRGFWPYAEMQNKIEFKLKQYGIEIRKVAPNNTSKTCSKCGHLNNYFNFEYRKMNKFPHFKCEKCNFKENADYNAALNISNPKLKSTKGEP

SEQ ID NO: 636 - protein, 726 aa, synthetic construct
SEVEFSHEYWMRHALTLAKRARDGREVPVGAVLVLNNRVIGEGWNRAIGLHDPTAHAEIMALRQGGLVMQNYRLIDATLYVTFEPCVMCAGAMVHSRIGRVVFGVRNSKRGAAGSLMNVLDYPGMGHRVEITEGILADECAALLCDFYCMPRQVFNAQKRARSCINSGGSSGGSSGSDTPGTSESATPESSGGGSSGSAKNTITKALKLRIVRPYNSAEVEKIVADEKNSREKIALEKNKGKVKEACSKHLKVAAYCTTQVERNACLFCKARKLDDKFYQKLRGQFPDAVFWQEIGEIFRQLQRQAAEIYNQSLIELYYEIFIKGKGFANASSVEHYLSDVCYTRAAELFKNAAIASGLRGKVKSNFRLKELKNMKSGLPTTKSDNFPIPLVKQKGGQYTGFEISSHNDDFIIKIPFGRWQVKKEIDKYRPWEKFDFEQVRKSPKPISLLLSTQRRKRNKGWSKDEGTEAEIRKVMNGDYQTSYIEVKRGSKTGEKSAWVLNLSIDVPKIDKGVDPSTIGGIDVGVKSPLVCAINNAFSRYSISDNDLFRFNKKMFARRRILLKKSKHKRAGHGAKNKLKPITILTEKSRRFRKKLIERWACEIADFFIKNKVGTVQMENLESMKRKEDSYFNIRLRGFWPYAEMQNKIEFKLKQYGIVVRKVAPNNTSKTCSQCGHLNNYFNFEYRKKNKFPYFKCEKCNFKENADYNAALNISNPQLKSTKGEP

SEQ ID NO: 637 - protein, 726 aa, synthetic construct
SEVEFSHEYWMRHALTLAKRARDEREVPVGAILVLNNRVIGEGWNRAIGLHDPTAHAEIMALRQGGLVMQNYRLTDATLYVTFEPCVMCAGAMIHGRIGRVVFGARNSKRGAAGSLMNVLNYPGMNHCVEITEGILVDECAALLCDFYHMPRQVLNAQKKAQSSISSGGSSGGSSGSETPGTSESATPESSGGGSSGSAKNTITKTLQLRIVRPYNSAEVEKIVADEKNNREKIALEKNKDKVKEACSKHLKMASYCTTQVERNACLFCKARKLDDKFYQKLRGQFPDAVFWQELGGIFRQLQKQAAEIYNQSLIELYYEIFIKGKGITNAGRVEHYLSDVCYTRAAELFKNAAIASGLRSKVRSNFRLKELKSMKSGLPTTKSDNFPIPLVKQKGGQYTGFEISSHNDDFIIKIPFGRWQVKKEIDKYRPWEKFDFEQVRKSPKPISLLLSTQRRKRNKGWSKDEGTEAEIRKVMNGDYQTSYIEVKRGSKTGEKSAWMLNLSIDVPKIDKGVDPCIIGGIDVGVKSPLVCAINNALSRYSISDNDLFHFNKKMFARRRILLRKNRHKRAGHGAKNKLKPITIMTERSKRFRKKLIERWACEIADFFIKNKVGTVQMENLESMKRREDSYFNIRLRGFWPYAEMQNKIEFKLKQYGIVVRKVAPNNTSKTCSKCGHLNNYFNFEYRKRNKFPHFKCEKCNFKENADYNAALNISNPKLKGTKEEP

SEQ ID NO: 638 - protein, 726 aa, synthetic construct
SEVEFSHEYWMRHALTLAKRARDEREVPVGAVLVLNNRIIGEGWNRAIGLHDPTAHAEIMALRQGGLVMQNYRLTDATLYVTFEPCVMCAGAMVHSRIGRVVFGVRNSKRGAAGSLMNVLNYPGVNHCVEITEGILVDECAALLCDFYRMPRQVLNAQKKAQSSISSGGSSGGSSGSETPGASGSVTPKSSVGSSGGSAKNTITKTLKLRIVRPYNSAEVEKIVTDEKNNREKIALEKNKDKVKEACSKHLKVASYCTTQVERNACLFCKARKLDDKFYQKLRGQFPDAVFWQELGGIFRQLQKQAAEIYNQSLIGLYYEIFIKGKGITNASRVEHYLSDVCYTRAAELFKNAAIASGLRSKVRSNFRLKELKNMKSGLPTTKSDNFPIPLVKQKGGQYTGFEISSHNNDFIIKIPFGRWQVKEEIDKYRPWEKFDFEQVRKSPKPISLLLSTQRRKKNKGWSKDEGTEAEIRRVMNGDYQTSYIEVKRGSKIGEKSAWMLNLSIDVPKIDKGVDPSIIGGIDVGVKSPLVCAINNAFSRYSISDNDLFHYNKKMFARRRILLKKNRHKRAGHGAKNKLKPISILTEKSKRFRKKLIERWACEIADFFIKNKVGTVQMENLESMKRKEDSYFNIRLRGFWPYAEMQNKIEFKLKQYGIEIRKVAPNNTSKTCSKCGHLNSYFNFEYRKRNGFPHFKCEKCNFKENADYNAALNISNPKLKSTKEEP

SEQ ID NO: 639 - protein, 726 aa, synthetic construct
SEVEFSHEYWMRHALTLAKRARDEREVPVGAVLVLNNRVIGVGWNRAIGLHDPTAHAEIMALRQGGLVTQNYRLIDATLYVTFEPCVMCAGAMIHSRIGRVVFGVRNSKHGAAGSLVNVLNYPGMNHRVEITEGILADECAALLCDFYRMPRQVFNARKKAQSSINSGGSSGGSSGSETPGTSESATPKSSGGSSGGSAKNTITKTLQLRIVRPYNSAEVEKIVADEKNNREKIALEKNKDKVKEACSKHLKVASYCTTQVERSACPFCKARKLDDKFYQKLRGQFPDAVFWQELGEILRQLQKQAAEIYNQSLIELYYEIFIKGKGFANASSVEHYLSDVCYTRAAELFKNAAIASGLRGKVKSNFRLKELKNMKSGLPTTKSDNFPIPLVKQKGGQYTGFEISSHNDDFIIKIPFGRWQMKKEIDRYRPWEKFDFEQVRRSPKPISLLLSTQRRKRNKGWSKDEGTEAEIRKVMNGDYQTSYIEVKRGSKIGEKSAWMLSLSIDVPKIDKGVDPSIIGGIDVGVKSPLVCAINNAFSRYSISDNDLFRFNKKMFARRRILLKKNRHKRAGHGARNKLKPITVLTEKSERFRKKLIERWACEIANFFIKNKVGTVQMENLESMKRREDSYFNIRLRGFWPYAEMQSKIEFKLKQYGIEIRKVAPNNTSKTCSKCGHLNSYFNFEYRKKNKFPHFKCEKCNFKENADYNAALNISNPRLKSTKEEP

SEQ ID NO: 640 - protein, 726 aa, synthetic construct
SEVEFSHEYWMRHALTLAKRARDEREVPVGAVLVLNNRVIGEGWNRAIGLHDPTAHAEIMALRQGGLVMQNYRLVDATLYVTFEPCVLCAGAMVHSRIGRVVFGVRNSKRGAAGSLMNVLNYPGMNHRVEITEGILADECAALLCDFYRMPRQVFNAQKKARSNINSGGSSGGSSGSETPGTSESATPVSSSGSSGGSAKDTITKTLKLRVVRPYNSAEVEKIVADEKNNREKIALAKNKDKVKEACSEHLKVAAYCTTQVERNACLFCKARKLDDKFYQKLRGQFPDAVFWQEIGEVFRQLQKQAAEIYNQSLIELYYEIFIKGKGFANASSVEHYLSDVCYTRAAELFKNAAIASGLRGKVKSNFRLKELKNMKSGLPTTKSDNFPIPLVKQKGGQYTGFEISSHNDDFIIKIPFGRWQVKKEINKFRPWEKFDFEQVRKSPKPLSLLLSTQRRKRNKGWSKDEGTEAEIRKVMNGDYQISYIEVKRGSKIGEKNAWMLNLSIDVPKIDKGVDPSIIGGIDVGVKSPLVCAINNAFSRYSISDNDLFRFNKKLFARRRILLKKNRHKRAGHGAKNKLKPISILTEKSKRFRKKLIERWACEIADFFIKNKVGTVQMENLESMKKKEDSYFNIRLRGFWPYAEMQNKIEFKLKQYGIEIRKVAPNNTSKTCSKCGHLNNYFNFEYRKKNKFPHFKCEKCNFKENADYNAALNISNPKLKSTKEGP

SEQ ID NO: 641 - protein, 726 aa, synthetic construct
SEVEFSHEYWMRHALTLAKRARDEREVPVGAVLVLNNRVIGEGWNRAIGLHDPTAHAEIMALRQGGLVMQNYRLSDATLYVTFEPCVMCAGAMIHSRIGRVVFGVRNSKRGAAGSLMNVLNYPGMNHCVEITEGILVDECVALLCDFYRMPRQVLSAQKKAQSSVSSGGSSGGSSGSETPGASGSVTPKSSGGSSAGSTKDTITKTLKLRIVRPYNSAEVEKIVADEKNSREKIALEKNRDKVKEACSEHLKVAVYCTTQVERNACLFCKARRLDDKFYQKLRGQFPDAVFWQEIGEIFRQLQKQAAEIYNQSLIELYYEIFIKGKGFANASSVEHYLSDVCYTRAAELFKNAAIASGLRGKVKSNFRLKELKNMKSGLPTTKSDNFPIPLVKQKGGQYTGFEISSHNDDFIIKIPFGRWQVKKEICKHRPWEKFDFEQVRKSPKPISLLLSTQRRKRNKGWGKDEGTEAEIRKVMNGDYQTSYIEVKRGSRIGEKSAWMLNLSIDVPKIDKGVDPSIIGGIDVGVKSPLVCAINNALSRYSISDNDLFHFNKKMFARRRILLRKNRHKRAGHGARNKLKPITVLTEKSERFRKKLIERWACEIANFFIKNKVGTVQMENLESMKRREDSYFNVRLRGFWPYAEMQSKIEFKLKQYGIKIRKVAPNNTSRTCSECGHLNNYFSFEYRKKNKFPHFKCKKCNFKEDADYNAALNISNPKLKGTKEEL

SEQ ID NO: 642 - protein, 726 aa, synthetic construct
SEVEFSHEYWMRHALTLAKRARDEREVPVGAVLVLNNRVIGEGWNRAIGLHDPTAHAEIMALRQGGLVMQNYRLTDATLYVTFEPCVMCAGAMVHSRIGRVVFGVRNSKRGAAGSLMNVLDYPGMGHRVEITEGILVDECAALLCDFYRMPRQVFNAQRKAQSNINSGGSSGGSSGSETPGTSESATLESSGGSSGGSAKNTITKTLKLRIVRPYNSTEVEKIVADEKNNREKIALEKNKDRVKEACSKHLKVASYCTTQVERNACLFCKARKLDDKFYQKLRGQFPDAVFWQELGEIFRQLQKQAAEIYNQSLIELYYEIFIKGKGFANASSVEHYLSDVCYTRAAELFKNAAIASGLRSKVRSNFRLKELKNMKSGLPTTKSDNFPIPLVKQKGGQYTGFEISSHNSDFIIKIPFGRWQVKEEIDKYRPWERFDFEQVRKSPKPISLLLSTQRRKRNKGWNKDEGTEAEIRKVMNGDYQTSYIEVKRGSKIGEKSAWMLNLSIDVPKIDKGVDPSIIGGIDVGVKSPLVCAINNAFGRYSISDNDLFHFNKKMFARRRILLKKNGHKRAGHGAKNKLKPITILTEKSKRFRKKLIERWASEIADFFIKNKVGTVQMENLESMKRKEDSYFNIRLRGFWSYAEMQNKIEFKLKQYGVEIRKVAPNNTSKTCSKCGHLNDYFNFEYRKKNKFPHFKCEKCNFKEDADYNAALNISNPKLKSTKEEH

SEQ ID NO: 643 - protein, 726 aa, synthetic construct
SEVEFSHEYWMRHALTLAKRARDEREVPVGAVLVLNNRVIGEGWNRAIGLHDPTAHAEIMALRQGGLVMQNYRLTDATLYVTFEPCVMCAGAMIHSRIGRVVFGVRNSKRGAAGSLMNVLNYPGMNHCVEITEGILVDECAALLCDFYRMPRQVLSAQKKAQSSISSGGSSGGSSGSETPGASGSVTPKSSVGSSAGSTKNTITKTLKLRIVRPYNSAEVEKIVADEKNNREKIALEKNKDKVKEACSKHLKVAAYCTTQVERNACLFCKARKLDDKFYQKLRGQFPDAVFWQEIGEIFRQLQKQAAEIYNQSLIELYYEIFIKGKGFANASSVEHYLSDVCYTRAAELFKNAAIASGLRGKVKSNFRLKELKNMKSGLPTTKSDNFPIPLVKQKGGQYTGFEISSHNDDFIIKIPFGRWQAKKEIDKYRPWEKFDFEQVRKSPKPISLLLSTQRRKRNKGWSKDEGTEAEIRKVMNGDYQTSYIEVKRGSKIGEKSAWMLNLSIDVPKIDKGVDPSIIGGIDVGVKSPLVCAINNAFSRYSISDNDLFHFNKKMFARRRILLKKNRHRRAGHGAKNKLKPISILTEKSKRFRKKLIERWACEIADFFIRNKVGTVQMENLEGMKRKEDSYFNIRLRGFWPYAEMQNKIEFKLKQYGIMVRKVAPNNTSKTCSKCGHLNNYFNFEYRKKNKFPHFKCEKCNFREDADYNAALNISNPKLKSTKEEP

SEQ ID NO: 644 - protein, 726 aa, synthetic construct
SEVEFSHEYWMRHALTLAKRARDEREVPVGAILVLHNRVIGVGWNRAIGLHDPTAHAEIMALRQGGLVMQNYRLIDATLYVTFEPCVMCAGAMIHSRIGRVVFGVRNSKHGAAGSLVNVLNYPGMNHRVEITEGILADECAALLCDFYRMPRQVFNARKKAQSSINSGGSSGGSSGSETPGTSESATPKSSSGSSGGSAKNTITKALKLRIVRPYNSAEVEKIVADEKNNRERIALEKNKDKVKEACSKHLKVAAYCTTQVERNACLFCKARKLDDKFYQKLRGQFPDAVFWQEIGEIFRQLQKQAAEIYNQSLIELYYEIFIKGKGFANAGSVEHYLSDVCYTRAAELFKNAAIASGLRGKVKSNFRLKELRNMKSGLPTTKSDNFPIPLVKQKGGQYTGFEISNHNGDFIIKIPFGRWQAKKEIDKYRPWEKFDFEQVRKSPKPISLLLSTQRRKRNRGWSKDEGTEAEIRKVMNGDYQTSYIEVKRGSKIGEKSAWMLNLSIDVPKIDKGVDPSIIGGIDVGVKSPLVCAINNTFSRYSISDNDLFRFNKKMFARRRILLGKNRHKRAGHGVKNKLKPITVLTEKSGRFRKKLIERWACEIADFFIKNKVGTVQMEDLESMKRREDSYFNIRLRGFWPYAEMQNKIEFKLKQYGIKIRRVAPNNTSKTCSKCGHLNNYFSFEYRKKNKFPHFKCEKCNFKENADYNAALNISNPKLMSTKEEP

SEQ ID NO: 645 - protein, 726 aa, synthetic construct
SEVEFSHEYWMRHALTLAKRARDEREVPVGAVLVLNNRVIGEGWNRAIGLHDPTAHAEIMALRQGGLVMQNYRLTDATLYVTFEPCVMCAGAMIHSRIGRVVFGVRNSKRGAAGSLMNVLNYPGMNHCVEITEGILMDECAALLCDFYRMPRQVFSARKKAQSSINPGGSSGGSSGSKTPGTSESATPGSSGGSSGGSAKNTITKTLKLRIVRPHNSAEVEKIVADEKNNREKIALEKNKGKVKEACSKHLEVAAYCTTQVERNACLFCKARKLDDKFYQRLRGQFPDAVFWQEIGEIFRQLQKQAAEIYNQSLIELYYEIFIKGKGFANASSVEHYLSDVCYTRAAELFKNAAIASGLRGKVKSNFRLKELKNMKSGLPTTKSDNFPIPLVKQKGGQYTGFEISSHNDDLIIKIPFGRWQVKKEINKYRPWEKFDFEQVRKSPKPISLLLSTQRRKRNKGWSKDEGTEAEIRRVMNGDYQTSYIEVKRGSKIGEKSAWMLNLSIDVPKIDKGVDPSIIGGIDVGVKSPLVCAINNAFSRYSISDNDLFRFNKKVFARRRILLKKNRHKRAGHGTKNKLKPITILTEKSGRFRKKLIERWACEIANFFIKNKVGTVQMENLESMKRKEDSYFNIRLRGFWPYAEMQNKIEFKLKQYGIKIRRVAPNNTSKTCSKCGHLNNYFSFEYRKKNKFPHFKCEKCNFKEDADYNAALNISDPKLKSTKEEP

SEQ ID NO: 646 - protein, 726 aa, synthetic construct
SEVEFSHEYWMRHALTLAKRARDEREVPVGAVLVLNNRVIGEGWNRAIGLHDPTAHAEIMALRQGGLVMQNYRLTDATLYVTFEPCVMCAGAMVHSRIGRVVFGVRNSKRGAAGSLMNVLNYPDMNHCVEITEGILVDECAALLCDFYRMPRQVLNAQKKARSSISSGGSSGGSSGSETPGASESVTPKSSGGSSGGSAKNTITKTLKLRIVRPYNSAEVEKIVADEKNNREKIALEKNKGKVKEACSKHLEVAAYCTTQVERNACLFCKARKLDDKFYQKLRGQFPDAVFWQELGEIFRQLQKQAAEIYNQSLIELYYEIFIKGKGLANASSVEHYLSDVCYTRAAELFKNAAIASGLRGKVKSNFRLKELKNMKSGLPTTKSDNFPIPLVKQKGGQYTGFEISSHNDDFIIKIPFGRWQVKKEIDKYRPWEKFDFEQVRKSPKPISLLLSTQRRKRNKGWSKDEGTEAEIRKVMNGDYQTSYIEVKRGSKTGEKSAWVLNLSIDVPKIDKGVDPSIIGGIDVGVKSPLVCAINNAFSRYSISDNDLFRFNKKVFARRRILLKKNRHKRAGHGAKNKLKPISILTGKSERFRKKLIERWACEIADFFIKNKVGTVQMENLESMKRKEDSYFNIRLRGFWPYAEMQNKIEFKLKQYGIEIRKVAPNNTSKTCSKCGHLNNYFNFEFRKKNKFPHFKCEKCNFKENADYNAALNISNPKLKSTKEEP

SEQ ID NO: 647 - protein, 726 aa, synthetic construct
SEVEFSHEYWMRHALTLARRARDEREVPVGAVLVLNNRVIGEGWNRTTGLHDPTAHAEIMALRQGGLVMQNYRLIDATLYVTFEPCVMCAGAMIHSRIGRVVFGVRNSKHGAAGSLVNVLNYPGMNHRVEITEGILADECAALLCDFYRMPRQVFNARKKTQSSINSGGLSGGSSGSDTPGTSESATPKSSGGSSGGSAKNTITKALKLRIVRPYNSAEVEKIVADEKNNRERIALEKNKDKVKEACSKHLKVAAYCTTQVERNACLFCKARKLDDKFYQKLRGQFPDAVFWQEIGEIFRQLQKQAAEIYNQSLIELYYEIFIKGRGFANASSVEHYLSDVCYTRAAELFKNAAIASGLRGKVKSNFRLKELKNMKSGLPTTKSDNFPIPLVKQKGGQYTGFEISSHNDDFIIKIPFGRWQAKKEIDKYRPWEKFDFEQVRKSPKPISLLLSTQRRKRNKGWSKDEGTEAEIRKVMNGDYQTSYIEVKRGSKIGEKSAWMLSLSIDVPKIDKGVDPSIIGGIDVGVKSPLVCAINNAFSRYSISDNDLFRFNKKMFARRRILLGKNRHKRAGHGVKNKLKPITILTEKSERFRKKLIERWACEIANFFIKNKVGTVQMENLESMKRREDSYFNIRLRGFWPYAEMQNKIEFKLKQYGIKIRKVAPNNTSKTCSKCGHLNNYFNFEFRKKNKFPHFKCERCNFKENADYNAALNISDPKLKSTKEES

SEQ ID NO: 648 - protein, 726 aa, synthetic construct
SEVEFSHEYWMRHALTLAKRARDEREVPVGAVLVLNNRVIGVGWNRAIGLHDPTAHAEIMALRQGGLVMQDYRLTDATLYVTFEPCVMCAGAMIHSRIGRVVFGVRNSKRGAAGSLMNVLNYPGMNHCVEITEGILVDECAALLCDFYRMPRQVLNAQKKAQSSISSGGSSGGSSGSETPGASGSVTPKSSGGSSTGSTKNTITKTLKLRIVRPYNSAEVEKIVADEKNSREKIALEKNKDKVKEACSEHLKVAAYCTTQVERNACLFCKARKLDDRFYQKLRGQFPDAVFWQEIGEIFRQLQKQAAEIYNQSLIELYYEIFIKGKGFAIASSVEHYLSCVCYTRAAELFKNAAIASGLRGKVKSNFRLKELKNMKSGLPTTKSDNFPIPLVKQKGGQYTGFEISSHNDDFIIKIPFGRWQVKKEIDKYRPWEKFDFEQVRKSPKPISLLLSTQRRKRNKGWSKDEGTEAEIRKVMNGDYQTSYIEVKRGGKIGEKSAWMLNLSIDVPKIDKGVDPSIIGGIDVGVKSPLVCAINNAFSRYSISDNDLFHFNKKMFARRRILLKKNRHKRAGHGVKNKLKPISILTEKSKRFRKKLIERWACEIADFFIKNKVGTVQMENLESMKRKEDSYFNIRLRGFWPYAEMQNKIEFKLKQYGIEIRKVAPNNTSKTCSKCGHLNNYFNFEYRRKNKFPHFKCEKCNFKEDADYNAALNISNPKLKSTKEEP

SEQ ID NO: 649 - protein, 726 aa, synthetic construct
SEVEFSHEYWMRRALTLAKRARDEREVPVGAVLVLNNRVIGEGWNRAIGLHDPTAHAEIMALRQGGLVMQNYRLVDATLYVTFEPCVLCAGAMVHSRIGRVVFGVRNNKRGAAGSLMNILNYPGMNHRVEITEGILADECAALLCDFYRMPRQVFSARKKAQSSINSGGSSGGNSGNKTPGTSESATPESSGGSSGGSAKNTITKTLKLRIVRPYNSAEVEKIVADEKNNREKIALEKNKDKVKEACSKHLKVASYCTTQVERNACLFCKARKLDDKFYQKLRGQFPDAVFWQEIGEIFRQLQKQAAEIYNQSLIELYYEIFIKGRGFANASSVEHYLSDVCYTRAAELFKNAAIASGLRGKVKSNFRLKELKNMKSGLPTTKSDNFPIPLVKQKGGQYTGFEISSHNDDFIIKIPFGRWQAKKEIDKYRPWEKFDFEQVRKSPKPISLLLSTQRRKRNKGWSKDEGTEAEIRRVMNGDYQTSYIEVKRGSKIGEKSAWMLNLSIDVPKIDKGVDPCIIGGIDVGVKSPLVCAINNASSRLSISDNDLFRFNKKMFARRRILLKKNGHKRAGHGAKNKLKPITILTEKSVRFRKKLIERWACEIADFFIRNRVGTVQMENLESMKRKEDSYFNIRLRGFWPYAEMQNKIEFKLKQYGIEIRKVAPNNTSKTCSKCGHLNNYFNFEYRKKNKFPHFKCEKCNFKENADYNAALNISNPKLRSTKEEP

SEQ ID NO: 650 - protein, 726 aa, synthetic construct
SEVEFSHEYWMRHALTLAKRARDEREVPVGAVLVLNNRVIGEGWNRAIGLHDPTAHAEVMALRQGGLVMQNYRLTDATLYVTFEPCVMCAGAMIHSRIGRVVFGVRNSKRGAAGSLMNVLNYPGMNHRVEITEGILVDECAALLCDFYRMPRQVLNAQKKAQSSISSGGSSGGSSGSETPGASGSVTPKSSGGSSAGSTKDTITKTLKLRIVRPYNSAEVEKIVADEKNSREKIALEKNKDKVKEACSEHLKVASYCTTRVERNACPFCKARKLDDKFYQKLRGQFPDAVFWQELGEILRQLQKQAAEIYNQSLIELYYEIFIKGRGFANASGVEHYLSDVCYTRAAELFKNAAIASGLRGKVKSNFRLKELKNMKSGLPTTKSDNFPIPLVKQKGGQYTGFEISSHNDDFIIKIPFGRWQVKKEIDKYRPWEKFDFEQVRKSPKPISLLLSTQRRRRNKGWSKDEGTEAEIRKVMNGDYQTSYIEVKRGSKTGEKSAWMLNLSIDVPKIDKGVNPSIIGGVDVGVKSPLVCAINNAFSRYSISDNDLFRFNKKVFARRRILLKKNRHKRAGHGAKNKLKPISILTGKSERFRKKLIERWACEIADFFIKNKVGTVQMENLESMKRREDSYFNIRLRGFWPYAEMQNKIEFKLKQYGIEVRKVAPNNTSKTCSKCGHLNNYFNFEYRKKNKFPHFKCEKCNFKENADYNAALNISNPRLKSTKEEP

SEQ ID NO: 651 - protein, 726 aa, synthetic construct
SEVEFSHEYWMRHALTLAKRARDGREVPVGAVLVLNNRVIGEGWNRAIGLHDPTAHAEIMALRQGGLVMQNYRLIDATLYVTFEPCVMCAGAMVHSRIGRVVFGVRNSKRGAAGSLMNVLDYPGMGHRVEITEGILADECAALLCDFYCMPRQVFNAQKRAQSSINSGGSSGGSSGSDTPGTSESATPESSGGGSSGSAKNTITKTLQLRIVRPYNSAEVEKIVADEKNNREKIALEKNKDKVREACSKHLKVASYCTTQVERNACPFCKARKLDDKFYQKLRGQFPDAVFWQELGEILRQLQKQAAEIYNQSLIELYYEIFIKGRGFANASSVEHYLSDVCYTRAAELFKNAAIASGLRGKVKGNFRLKELKNMKSGLPTTKSDNFPIPLVKQKGGQYTGFEISSHNDDFIIKIPFGRWQAKKEIDKYRPWEKFDFEQVRKSPKPISLLLGTQRRKRNRGWSKDEGTEAEIRKVMNGDYQTSYIEVKRGSKIGEKSAWMLNLSIDVPKIDKGVDPSIIGGIDVGVKSPLVCAINNAFSRYSISDNDLFRFNKKMFARRRILLGKNRHKRAGHGVKNKLKPITILTEKSGRFRKKLIERWACEIADFFVKNKVGTVQMENLESMKRKEDSYFNIRLRGFWPYAEMQNKIEFKLKQYGIEIRKVAPNNTSKTCSKCGHLNNYFNFEYRKKNKFPHFKCEKCNFKENADYNAALNISNPKLKSTKEEP

SEQ ID NO: 652 - protein, 726 aa, synthetic construct
SEVEFSHEYWMRHALTLAKRARDEREVPVGAVLVLNNRVIGEGWNRAIGLHDPTAHAEIMALRQGGLVMQNYRLIDATLYVTFEPCVMCAGAMIHSRIGRVVFGVRNSKHGAAGSLMNVLNYPGMNHRVEITEGILVDECAALLCDFYRMPRQVFNARKKAQSSIDPSGSSGGSSGSVTPGTSESATPESSGGGFGGSAKNTITKTLQLRIVRPYNSAEVEKIVADEKNNREKIALEKNKDKVKEACSKHLKVASYCTTQVERNACLFCKARKLDDRFYQKLRGQFPDAVFWQELGEIFRQLQKQAAEIYNQSLIELYYVIFIKGKGLANASSVEHYLSDVCYTRAAELFKNAAIASGLRGKVKSNFKLKELKSMKSGLPSTKSDNFPIPLVKQKGGQYTGFEISSHNDDLIIKIPFGRWQVKKEIDKYRPWEKFDFEQVRKSPKPISLLLSTQRRKRNKGWGKDEGTEAEIRKVMNGDYQTSYIEVKRGSKIGEKSAWMLNLSIDVPKIDKGVDPSIIGGIDVGVKSPLVCAINNAFSRYSISDNDLFRFNKKMFARRRILLKKNRHKRAGHGAKNKLKPISILTERSERFRKKLIERWACEIADFFIKNKVGTVQMENLESMKRKEDSYFNIRLRGFWPYAEMQNKIEFKLKQYGIEIRKVAPNNTSKTCSKCGHLNNYFNFEYRKKNKFPHFKCEKCNFKENADYNAALNISNPKLKSTKGEP

SEQ ID NO: 653 - protein, 726 aa, synthetic construct
SEVEFSHEYWMRHALTLAKRARDEREVPVGAVLVLDNRVIGEGWNRAIGLHDPTAHAEIMALRQGGLVMQNYRLTDATLYVTFEPCVMCAGAMIHSRIGRVVFGVRNSKRGAAGSLMNVLNYPGMNHCVEITEGILMDECAALLCDFYRMPRQVLNAQKKAQSSISSGGSSGGSSSSETPGASESVTPKSSVGSSAGSTKNTITKTLKLRIVRPYNSAEVEKIVADEKNNRERIALEKNKDKVKEACSKHLKVAAYCTTQVERNACLFCKARKLDDKFYQKLRGQFPDAVFWQEIGEIFRQLQKQAAEIYNQSLIELYYEILIKGKGFANASSVEHYLSDVCYTRAAELFKNAAIASGLRGKVKSNFRLKELKNMKSGLPTTKSDNFPIPLVKQKGGQYTGFEISSHNDDFIIKIPFGRWQAKKEIDKYRPWEKFDFEQVRKSPKPISLLLSTQRRKRNKGWSKDEGTEAEIRKVMNGDYQTSYIEVKRGSRTGEKSAWMLNLSIDVPKIDKGVDPSIIGGIDVGVKSPLVCAINNAFSRYSISDNDLFRFNKKMFARRRILLKKNRHKRAGHGAKNKLKPISILTGKSERFRKKLIERWACEIADFFIKNKVGTVQMENLESMKRKEDSYFNIRLRGFWPYAEMQNKIEFKLKQYGIEIRKVAPNNTSKTCSKCGHLNNYFNFEYRKKNKFPHFKCEKCNFKENADYNAALNISNPKLKSTKEEP

SEQ ID NO: 654 - protein, 726 aa, synthetic construct
SEVEFSHEYWMRHALTLAKRARDEREVPVGAVLVLNNRVIGEGWNRTTGLHDPTAHAEIMALRQGGLVMQNYRLVDATLYVTFEPCVLCAGAMVHSRIGRVVFGVRNSKRGAAGSLMNVLDYPGMNHRVEITEGILADECAALLCDFYRMPRQVFNAQKKARPNINSGGSSGGRSGSETPGTSESATPESSGGSSGGSAKNTITKTLKLRIVRPYNSAEVEKIVADEKNNREKIALEKNKDKVKEACSKHLKVAAYCTTQVERNACLFCKARKLDDGFYQKLRGQFPDAVFWQEIGEILRQLQKQAAEIYNQSLIELYYEIFIKGRGFANASSVEHYLSDVCYTRAAELFKNAAIASGLRGKVKSNFRLKELKNMKSGLPTTKSDNFPIPLVKQKGGQYTGFEISSHNDDFIIKIPFGRWQVKKEIDKYRPWEKFDFEQVRKSPKPISLLLSTQRRKRNKGWSKDEGTEAEIRKVMNGDYQTSYIEVKRGSKIGEKSAWMLNLSIDVPKIDKGVDPSIIGGIDVGVKSPLVCAINNAFSRYSISDNDLFRYNKKMFARRRILLKKNRHKRAGHGTKNKLKPITILTEKSRRFRKKLIERWACEIADFFIKNKVGTVQMESLESMKRKEDSYFNIRLRGFWPYAEMQNKIEFKLKQYGIKIRKVAPNNTSKTCSMCGHLNNYFSFEYRKKNKFPHFKCEKCNFKENADYNAALNISNPKLMSTKEGP

SEQ ID NO: 655 - protein, 726 aa, synthetic construct
SEVEFSHEYWMRHALTLAKRARDEREVPVGAVLVLNNRVIGEGWNRAIGLHDPTAHAEIMALRQGGLVMQNYRLTDATLYVTFEPCVMCAGAMIHSRIGRVVFGVRNSKRGAAGSLMNVLNYPGMNHCVEITEGILVDECAALLCDFYRMPRQVLNAQKKAQSSISSGGSSGGSSCSETPGASESVTPKSSGGSSAGSTKNTITKTLKLRIVRPYNSAEVEKIVADEKNNREKIALEKNKDKVKEACSKHLKVATYCTTQVGRNACLFCKARKLDDKFYQKLRGQFPDAVFWQEIGEIFRQLQKQAAEIYNQSLIELYYEIFIKGKGFANASSVEHYLSDVCYTRAAKLFKNAAIASGLRGKVKSNFRLKELKNMKSGLPTTKSDNFPIPLVKQKGGQYTGFEISSHNDDFIIKIPFGRWQVKKEIDKYRPWEKFDFEQVRKSPKPISLLLSTQRRKRNRGWSKDEGTEAEIRKVMNGDYQTSYIEVKRGSKIGEKSAWMLNLSIDVPKIDKGVDPSIIGGIDVGVKSPLVCAINNAFSRHSISDNDLFHFNKKMFARRRILLKKNRHKRAGHGAKNKLKPISILTERSKRFRKKLIERWACEIADFFIKNKVGTVQMENLESMKRKEDSYFNIRLRGFWPYAEMQNKIEFKLKQYGIEIRKVAPNNTSKTCSKCGHLNNYFNFEYRKRNKFPHFKCEKCNFKENADYNAALNISNPKLKSTKEEP

SEQ ID NO: 656 - protein, 726 aa, synthetic construct
SEVVFSHEYWMRHALTLAKRARDEREVPVGAVLVLNNRVIGEGWNRAIGLHDPTAHAEIMALRQGGLVMQNYRLTDATLYVTFEPCVMCAGAMIHSRIGRVVFGVRNSKRGAAGSLMNVLNYPGTNHCVEITEGILVDECAALLCDFYRMPRQVLNAQKKAQSSISSGGSSGGSSCSETPCASESVTPKSSGGSSAGSTKNTITKTLKLRIVRPYNSAEVEKIVADEKNSREKIALEKNKDKVKEACSEHLKVAAYCTTQVERNACLFCKARKLDDRFYQKLRGQFPDAVFWQEIGEIFRQLQKQAAEIYNRSLIELYYEIFIKGKGFANASSVEHYLSDVCYTRAAELFKNAAIASGLRGKVKSNFRLKELKNMKSGLPTTKSDNFPIPLVKQKGGQYTGFEISSHNDDFIIKIPFGRWQVKKEINKFRPWEKFDFEQVRKSPKPISLLLSTQRRKRNKGWGKDEGTEAEIRKVMNGDYQTSYIEVKRGSKTGEKSAWMLNLSIDVPKIDKGVDPSIIGGIDVGVKSPLVCAINNAFSRYSISDNDLFRFNKRMFARRRILLKKNRHKRAGHGAKNKLKPISILTGKSERFRKKLIERWACEIADFFIKNKVGTVQMENLESMKRKEDSYFNIRLRGLWPYAEMQNKIEFKLKQYGIKIRKVAPNNTSKTCSKCGHLNNYFNFEYRKKNKFPHFKCEKCSFKENADYNAALNISNPKLKSTKEEP

SEQ ID NO: 657 - protein, 726 aa, synthetic construct
SEVEFSHEYWMRHALTLAKRARDKHEVPVGAVLVLDNRVIGEGWNRATGQNDPTAHAEIMALRQGGLVMQNHRLIDATLYVTFEPCVMCAGAMIHSRIGRVVIGVRNSKRGAAGSLMNVLNHPGMNHRVEITEGILADECAALLCDFYRMPRRVFNAQRKAQSSINSGGSPGGGSGSDTPSTSESTTPESSGGSSGGPAKNTITKTLKLRIVRPYNSAEVEKIVADEKNNREKTALEKNKDKVKEACSKHLKVASYCTTQVERNACLFCKARKLDDKFYQKLRGQFPDAVFWQELGEIFRQLQKQAAEIYNQSLIELYYEIFIKGKGVANASGVEHYLSDVCYTRAAELFKNAAIASGLRSKVKSNFRLKELKNMKSGLPTTKSDNFPIPLVKQKGGQYTGFEISDHNSDFIIKIPFGRWQVKKEIDKFRPWEKFDFEQVRKSPKPISLLLSTQRRKRNKGWSKDEGTEAEIRKVMNGVYQTSYIEVKRGSKIGEKSAWMLNLSIDVPKIDKGVDPSIIGGIDVGVKSPLVCAINNAFSRYSISDNDLFHFNKKMFARRRILLKKNRHRRAGHGAKNKLKPIAVLAEKSEGFRKKLIERWACEIADFFVKNKVGTVQMENLESMKRKEDSYFNIRLRGFWPYAEMQNKIEFKLKQYGIKVRKVAPNNTSKTCSKCGHLNNYFSFEYRKKNKFPHFKCEKCNFKENADYNAALNISNPKLKSTKEEP

SEQ ID NO: 658 - protein, 726 aa, synthetic construct
SEDEFSHEYWMRHALTLAKRARDGREVPVGAVLVLNNRVIGEGWNRAIGLHDPTAHAEIMALRQGGLVMQNYRLIDATLYVTFEPCVMCAGAMVHSRIGRVVFGVRNSKRGAAGSLMNVLDYPGMGHRVEITEGILADECAGLLCDFYCMPRQVFNAQKRAQSSINSGGSSGGSSGGDTPGTSESATPESSGGGSSGSAKNTTTKTLQLRIVRPYNSAEVEKIVADEKNNREKIALEKNKDKVREACSKHLKVASYCTTQVERNACPFCKARKLDDKFYQKLRGQFPDAVFWQELGEILRQLQKQAAEIYNRSLIELYYEIFIKGRGFANASSVEHYLSDVCYTRAAELFKNAAIASGLRGKVKGNFRLKELKNMKSGLPTTKSDNFPIPLVRQKGGQYTGFEISSHNDDFIIKIPFGRWQVKKEIDKYRPWEKFDFEQVRKSPKPISLLLSTQRRKRNKGWSKDEGTEAEIRKVMNGDYQTSYIEVKRGSKIGEKSAWMLNLSIDVPKIDKGVDPSIIGGIDVGVRSPLVCAINNAFSRYSISDNDLFRFNKKMFARRRILLKKNRHKRAGHGAKNKLKPITTLTEKSRRFRKKLIERWACEIADFFIKNKVGTVQMESLESMKRREDSYFNVRLRGFWPYAEMQNKIEFKLKQYGIKIRKVAPNNTSKTCSMCGHLNNYFSFEYRKKNKFPHFKCKKCNFKEDADYNAALNISNPKLKSTKEKP

SEQ ID NO: 659 - protein, 726 aa, synthetic construct
SEVEFSHEYWMRHALTLAKRARDEREVPVGAVLVLNNRVIGEGWNRAIGLHDPTAHAEIMALRQGGLAMQNYRLVDATLYVTFEPCVLCAGAMVHSRIGRVVFGVRNSKRGAAGSLMNVLNYPGMNHRVEITEGILADECAALLCDFYRIPRRVFNAQKKAQSNINPGGSSGGSGGSETPGTSESATPKSSGGSSGGSAKNTITKTLKLRIVRPYNSAEVEKIVADEKNNREKIALEKNKGKVKEACSKHLEVAAYCTTQVERNACLFCKARKLDDKFYQKLRGQFPDAVFWQEIGEIFRQLQKQAAEIYNQSLIELYYEIFIKGKGFANASSVEHYLSDVCYTRAAELFKNAAIASGLRGKVKSNFRLKELKNMRSGLPTTKSDNFPIPLVKQKGGQYTGFEISSHNDDFIIKIPFGRWQVKKEIDKYRPWEKFNFEQVRKSPKPISLLLSTQRRKRSKGWSKDEGTEAEIRRVMNGDYQTSYIEVKRGSKIGEKSAWMLNLSIGVPKIDKGVDPSIIGGIDVGVKSPLVCAINNAFSRYSISDNDLFHFNKKVFARRRILLKKNRHKRAGHGAKNKLKPISILTEKSKRFRKKLIERWACEIADFFIKNKVGTVQMENLESMKRKEDSYFNIRLRGLWPYAEMQNKIEFKLKQYGIRIRKVAPNNTSKTCSKCGHLNNYFNFEYRKKNKFPHFRCEKCNFKENADYNAALNISNPKLKSTKEEP

SEQ ID NO: 660 - protein, 726 aa, synthetic construct
NEVEFSHEYWMRHALTLAKRARDEREVPVGAILVLNNRVIGEGWNRAIGLHDPTAHAEIMALHQGGLVMQNYRLIDATLYVTFEPCVMCAGAMIHSRIGRVVFGARNSKRGAAGSLMNVLSYPGMNHRVEITEGILADECAALLSDFYRMPRRVFNAQKKAQSSINSGGSSGGSSGSETPGASGSVTPKSSGGSSAGSAKDTITKTLKLRIVRPYNSAEVEKIVADEKNSREKIALEKNKDKVKEACSKHLKVAAYCTTQVERNACLFCKARKLDDKFYQKLRGQFPDAVFWQEVGEIFRQLQKQAAEIYNQSLIELYYEIFIKGKGFANASSVEHYLSDVCYTRAAELFKNAAIASGLRGKVKSNFRLRELKNMKSGLPTTKSDNFPIPLVKQKGGQYTGFEISSHNDDFIIKIPFGRWQVKKEIDKYRPWEKFDFEQVRKSPKPISLLLSTQRRKRNKGWSKDEGTEAEIRRVMNGDYRTSYIEVKRGSKTGEKSAWMLNLSIDVPKIDKGVDPSIIGGIDVGVKSPLVCAINNAFSRYSISDNDLFRFNKKMFARRRVLLKKNRHKRAGHGAKNKLKPISILTEKSKRFRKKLIERWACEIADFFIKNKVGTVQMENLESMKRKEDSYFNIRLRGFWPYAEMQNKIEFKLKQYGIEIRKVAPNNTSKTCSKCGHLNNNFNFEYRRKNKFPHFKCEKCNFKEDADYNAALNISNPKLKSTKEEP

SEQ ID NO: 661 - protein, 726 aa, synthetic construct
SEVEFSHEYWMRHALTLAKRARDEREVPVGAVLVLNNRVIGVGWNRAIGLHDPTAHAEIMALRQGGLVMQNYRLTDATLYVTFEPCVMCAGAMVHSRIGRVVFGVRNSKRGAAGSLMNVLNFPGMSHCVEITEGILVDECAALLCDFYRMPRQVLNAQKKAQSSISSGGSSGGSGGGETPGASESVTPKNSGGSSASSTKNTITKTLKLRIVRPYNSAEVEKIVADEKNSREKIALEKNKDKVKEACREHLKVAAYCTTQVERSACLFCKARKLDDRFYQKLRGQFPDAVFWQEISEIFRQLQKQAAEIYNQSLIELYYEVLIKGKGIANASRVEHYLSDVCYTRAAELFKNAAIASGLRGKVKSNFKLKELKSMKSGLPSTKSDNFPIPLVKQRGGQYTGFEISSHNDDFIIKIPFGRWQVKKEIDKYRPWEKFDFEQVRKSPKPISLLLSTQRRKRNRGWSKDEGTEAEIRKVMNGDYQTSYIEVKRGSKIGEKSAWMLNLSIDVPKIDKGVDPSIIGGIDVGVKSPLVCAINNALSRYSISDNDLFHFNKKMFARRRILLRKNRHKRAGHGAKNKLKPITIMTEKSKRFRKKLIERWACEIADFFVKNKVGTVQMENLESMKRKEDSYFNIRLRGFWPYAEMQNKIEFKLKQYGIEIRKVAPNNTSKTCSKCGHLNNYFNFEYRKMNKFPHFKCEKCNFKENADYNAALNISNPKLKSTKEEP

SEQ ID NO: 662 - protein, 726 aa, synthetic construct
SEVEFSHEYWMRHALTLAKRARVEREVPVGAVLVLNNRVIGEGWNRAIGLHDPTAHAEIMALRQGGLVMQNYRLIDATLYVTFEPCVMCAGAMIHSRIGRVVFGVRNSKHGAAGSLVNVLNYPGMNHRVEITEGILADECAALLCDFYRMPRQVFNAWKKAQSSINPSGSSGGSSGSVTPGTSESATPESSGGGFGGSAKNTITKTLQLRIVRPYNSAEVEKIVADEKNNREKIALEKNKDKVKEACSKHLKVAPYCTTQVERNACLFCKARKLDDRFYQKLRGQFPDAVFWQELGEIFRQLQKQAAEIYNQSLIELYYVIFIKGKGFANASSVEHYLSDVCYTRAAELFKNAAIASGLRGKVKSNFRLKELKNMKSGLPTTKSDNFPIPLVKQKGGQYTGFEISNHNDDFIIKIPFGRWQVKKEIDKYRPWEKFDFEQVRKSPKPISLLLSTQRRKRNKGWSKDEGTEAEIRKVMSGDYQTSYIEVKRGSKTGEKSAWMLNLSIDVPKIDKGVDPSIIGGIDVGVKSPLVCAINNAFSRYSISDNDLFRFNKKMFARRRILLKKNRHKRAGHGAKNKLKPITILTEKSGRFRKKLIERWACEIANFFIKNKVGTVQMENLESMKRKEDSYFNIRLRGFWPYAEMQNKIEFKLKQYGIKIRKVAPNNTSKTCSKCGHLNNYFSFEYRKKNKFPHFKCEKCNFKEDADYNAALNISNPKLKSTKEEP

SEQ ID NO: 663 - protein, 726 aa, synthetic construct
SEVEFSHEYWMRHALTLAKRARDEREVPVGAVLVLNNRVIGEGWNRAIGLHDPTAHAEIMALRQGGLVMQNYRLTDATLYVTFEPCVMCAGAMIHSRIGRVVFGVRNSKRGAAGSLMNVLNYPGMNHCVEITEGILVDECAALLCDFYRMPRQVLNAQKKARSSISSGGSSGGSSGSETPGASGSVTPKSSGGSSAGSTKDTITKTLKLRIVRPYNSAEVEKIVADEKNSREKNALEKNKDKVKEACSKHLKVAAYCTTQVERNACLFCKARRLDDKFYQKLRGQFPDAVFWQEIGEIFRQLQKQAAEIYNQSLVELYYEIFIKGKGIANASSVEHYLSDVCYTRAAELFKNAAIASGLRNKIKSNFRLKELRNMKSGLPTTKSDNFPIPLVRQKGGQYTGFEISNHNGDFIIKIPFGRWQVKKEISKHRPWEKFDFEQVRKSPKPISLLLSTQRRKRNKGWGKDEGTEAEIRKVMNGDYRTSYIEVKRGSKIGEKSAWMLNLSIDVPKIDKGVDPSIIGGIDVGVKSPLVCAINNALSRYSISDNDLFHYNKKMFARRRILLKKNRHKRAGHGARNKLKPISILTEKSKRFRKKLIERWACEIADFFIKNKVGTVQIENLESMKRKEDSYFNTRLRGFWPYAEMQNKIEFKLKQYGIEIRKVAPNNTSKTCSKCGHLNSYFNFEYRKKNKFPHFKCEKCNFRENADYNAALNISNPKLRSTKEEP

SEQ ID NO: 664 - protein, 726 aa, synthetic construct
SEVEFSHEYWMRHALTLAKRARDEREVPVGAVLVLNNRVIGEGWNRAIGLHDPTAHAEIMALRQGGLVMQNYRLVDATLYVTFEPCVMCAGAMIHSRIGRVVFGVRNNKHGAAGSLVNVLNYPGMNHRVEITEGILADECAALLCDFYRMPRQVFNARKKAQSSINPGGSSGGSSGSETPGTSESATPESSGGSSGSSAKNTITKTLKLRIVRPYNSAEVEKIVADEKNNREKIALEKNKDKVEEACSKHLKVAAYCTTQVERNACLFCKARRLDDKFYQKLRGQFPDAVFWQEIGEIFRQLQKQAAEVYNQSLVELYYEILIKGKGIANASSVEHYLSDVCYTRAAELFKNAAIASGLRNKIKSNFRLKELRNMKSGLPTTKSDNFPIPLVRQKGGQYTGFEISNHDGDFIIKFPFGRWQVKKEIDKYRPWEKFDFEQVRKSPKPISLLLSTQRRKRNKGWSKDEGTEAEIRKVMNGDYQTSYIEVKRGSKTGEKSAWMLSLSIDVPKIDKGVDPSIIGGIDVGVKSPLVCAINNAFSRYSISDNDLFRFNKKMFARRRILLKKNRHKRAGHGAKNKLKPISILTGKSERFRRKLIERWACEIADFFIKNKVGTVQMENLESMKRKEDSYFNIRLRGFWPYAEMQNKIEFKLKQYGIEIRKVAPNNTSKTCSKCGHLNNYFNFEYRRKNKFPHFKCEKCNFKENADYNAALNISNPKLKSTKEEP

SEQ ID NO: 665 - protein, 726 aa, synthetic construct
SEVEFSHEYWMRHALILAKRARDEREVPVGAVLVLNNRVIGVGWNRAIGLHDPTAHAEIMALRQGGLVMQNYRLIGATLYVTFEPCAMCAGAMIHSRIGRVVFGVRNSKRGAAGSLMNVLNYPGMNHRVEIMEGILTDECAALLCDFYRMPHQVLNAQKKAQSSINSGGSSGGSSGSETPGTSGSATPEGSGGSSGGSTKNTITKTLKLRIVRPYNSAEVEKIVADEKNNREKIALEKNKGKVKEACSKHLKVATYCTTQVERNACLFCKARKLDDKFYQKLRGQFPDAVFWQEVGEIFRQLQKQAAEIYNQSLIELYYEIFIKGKGIANASSVGHYLSDVCYTRAAELFKNAAIASGLRGKVKGNFRLKELKNMKGGLPTTKSDNFPIPLVKQKGGQYTGFEISSHNDDFIIKIPFGRWQVKKEIDKYRPWEKFDFEQVRKSPKPISLLLSTQRRKRNKGWSKDEGTEAEIRKVMSGDYQTSYIEVKRGSKTGEKSAWMLSLSIDVPKIDKGVDPSIVGGIDVGVKSPLVCAINNALGRYSISDNDLFHFNKKMFARRRILLKKNRHKRAGHGAKNKLKPITILTEKSVRFRKKLIERWACEIADFFIKNKVGTVQMENLESMKRKEDSYFNIRLRGFWPYAEMQNKIEFKLKQYGIEIRKVAPNNTSKTCSKCGHLNNYFSFEYRKKNKFPHFKCEKCNFKENADYNAALNISNPKLKSTKGEP

SEQ ID NO: 666 - protein, 726 aa, synthetic construct
SEVEFSHEYWMRHALTLAKRARDEREVPVGAILVLNNRVIGEGWNRAIGLHDPTAHAEIMALRQGGLVMQNYRLIGATLYVTFEPCVMCAGAMIHSRIGRVVFGVRNNKHGAAGSLVNVLNYPGMNHRVEITEGILADECAALLCDFYRMPRQVFNARKKAQSSINSGGSSGGSSGSETPGTSESATPESSGGGSSGSAKNTITKTLKLRIVRPYNSTEVEKIVADEKNNREKIALEKNKDKVKEACSKHLKVASYCTTQVERNACLFCKARKLDDKFYQKLRGQFPDAVFWQEIGEIFRQLQKQAAEIYNQSLIELYYEIFIKGKGFANASSVEHYLSDVCYTRAAGLFKNAAIASGLRGKVKSNFRLKELKSMKSGLPTTKSDNFPIPLVKQKGGQYTGFEISNHNSDFIIKIPFGRWQVKKEIDKYRPWEKFDFEQVRKSPKPISLLLSTQRRKRNKGWSKDEGTEAEIKRVMNGDYQISYIEVKRGSKIGEKSAWMLSLSVDVPKIDKGVDPSIIGGIDVGVKSPLVCAINNALSRYSISDNDLFHFNKKMFARRRILLRKNRHKRAGHGAKNKLKPITIMTEKSKRFRKKLIERWACEIADFFIKNKVGTVQMENLEGMKRKEDSYFNIRLRGFWPYAEMQNKIEFKLKQYGIEVRKVAPNNTSKTCSKCGHLNNYFNFEFRKKSKFPHFKCEKCNFKEDADYNAALNISNPKLKSTKEEP

SEQ ID NO: 667 - protein, 726 aa, synthetic construct
SGVEFSHEYWMRHALTLAKRARDEREVPVGAVLVLNNRVIGEGWNRAIGLHDPAAHAEIMALRQGGLVMQNYRLIGATLYVTFEPCVMCAGAMIHSRVGRVVFGVRNNKHGAAGSLVNVLNYPGMNHRVEITEGILADECAALLCDFYRMPRQVFNARKKAQSGINPGDSSGGSGGGETPGASESVTPKSSGGSSAGSTKSTITKTLKLRIVRPYNSAEVEKIVADEKNSREKIALEKNKDKVKEACSKHLKVASYCTTQVERNACPFCKARKLDDKFYQKLRGQFPDAVFWQELGEILRQLQKQAAEIYNQSLIELYYEIFIKGRGFANASSVEHYLSDVCYTRAAELFKNAAIASGLRGKVKSNFRLKELKNMKSGLPTTKSDNFPIPLVKQKGGQYTGFEISSHNDDFIIKIPFGRWQVKKEIDKYRPWEKFDFEQVRKSPKPISLLLSTQRRKRNKGWSKDEGTEAEVRKVMNGDYRTSYIEVKRGSKTGEKSAWMLNLSIDVPKIDKGVDPSIIGGIDVGVKSPLVCAINNAFSRYSISDNDLFRFNKKMFARRRILLKKNRHKRAGHGAKNKLKPISILTEKSKRFRKKLIERWACEIADFFIKNKVGTVQMENLESMKRKEDSYFNIRLRGFWPYAEMQNKIEFKLKQYGIEIRKVAPNNTSKTCSKCGHLNNYFNFEYRRKNKFPHFKCEKCNFKEDADYNAALNISNPKLKSTKEEP

SEQ ID NO: 668 - protein, 726 aa, synthetic construct
SEVEFSHEYWMRHALALAKRARDEREVPVGAILVLNNRVIGEGWNRAIGLHDPTAHAEIMALRQGGLVLQNYRLIDATLYVTFEPCVMCAGAMIHSRIGRVVFGVRNNKHGAAGSLVNVLNYPGMNHRVEITEGILADECAALLCDFYRMPRLVFNARKKTQSSINPGGSSGGSSGSETPGTSESPTPESSGGSSGSSAKNTITKTLKLRIVRPYNSAEVEKIVADEKNNREKIALEKNKDKVKEACSKHLKVAAYCTTQVERNACLFCKARKLDDKFYQKLRGQFPDAVFWQEIGEIFRQLQKQAAEIYNQSLIELYYEIFIKGKGFANASSVEHYLSDVCYTRAAELFKNAAIASGLRGKVKSNFRLKELKNMKSGLPTTKSDNFPIPLVKQKGGQYTGFEISSHNDDFIIKIPFGRWQVKKEINKYRPWEKFDFEQVRKSPKPISLLLSTQRRKRNRGWSKDEGTEAAIRKVMNGDYQTSYIEVKRGSKIGEKSAWMLNLSIDVPKIDKGVDPSIIGGIDVGVKSPLVCAINNAFSRYSISDNDLFRFNKKMFARRRILLGKNRHKRAGHGVKNKLKPITILTEKSGRLRKKLIERWACEIADFFVKNKVGTVQMENLESMKRKEDSYFNIRLRGFWPYAEMQNKIEFKLKQYGIKVRKVAPNNTSKTCSKCGHLNNYFSFEYRKKNKFPHFKCEKCNFKENADYNAALNISNPKLKSTKEEP

SEQ ID NO: 669 - protein, 726 aa, synthetic construct
SEVEFSHEYWMRHALTLAKRARDEREVPVGAVLVLNNRVIGEGWNRAIGLHDPTAHAEIMALRQGGLVMQNYRLADATLYVTFEPCVMCAGAMIHSRIGRVVFGVRNSKRGAAGSLMNVLNYPGMNHCVEITEGILVDECAALLCDFYRMPRQVLNAQKKAQSSISSGGSSGGSSGSETPGASESVTPKSSGGSSAGSTKNTITKTLQLRIVRPYNSAEVEKIVADEKNNRERIALEKNKDKVKEACSKHLKVAAYCTTQVERNACLFCKARKLDDKFYQKLRGQFPDAVFWQEIGEIFRQLQKQAAEIYNQSLIELYYEIFIKGKGFANASSVEHYLSDVCYARAAELFKNAAIASGLRGKVKSNFRLKELKNMKSGLPTTKSDNFPIPLVKQKGGQYTGFEISNHSDDFIIKIPFGRWQVKEEIDKYRPWEKFDFEQVRKNPKPISLLLSTQRRKRNKGWSKDEGTEAEIRKVMNGDYQTSYIEVKRGSKIGEKSAWMLNLSIDVPKIDKGVDPSIIGGVDVGVKSPLVCAINNAFSRYSISDNDLFRFNKRMFARRRILLKKNRHKRAGHGAKSKLKPISILTEKSERFRKKLIERWACEIADFFIKNKVGTVQMENLESMKRKEDSYFNIRLRGFWPYAEMQNKIEFKLKQYGIKIRKVAPNNTSKTCSKCGHLNNYFSFEYRKKNKFPHFKCEKCNFKEDADYNAALNISNPKLKSTKEEP

SEQ ID NO: 670 - protein, 726 aa, synthetic construct
SEVEFSHEYWMRHALTLAKRARDEREVPVGAILVLNNRVIGEGWNRAIGLHDPTAHAEIMALRQGGLVMQNYRLIDATLYVTFEPCVMCAGAMIHSRIGRVVFGVRNSKRGAAGSLMNVLNYPGMNHCVEITEGILADECAALLCDYYRMPRQVFNARKKAQSSINSGGSSDGGSGSETPGTSGSATPEGSGGSSGGSAKNTITKTLKLRIVRPYNSAEVEKIVADEKNNREKIALEKNKDKVKEACSKHLKVASYCTTQVERNACLFCKARKLDDKFYQKLRGQFPDAVFWQELGEIFRQLQKQAAEIYNQSLIELYYEIFIKGKGFANASSVEHYLSDVCYTRAAELFKNAAIASGLRGKVKSNFRLKELKNMKSGLPTTKSDNFPIPLVKQKGGQYTGFEIGSHNDDFIIKIPFGRWQVKKEIDKYRPWEKFDFEQVRKSPKPISLLLSTQRRKRNKGWSRDEGTEAEIKKVMNGDYQTSYIEVKRGSKTGEKSAWMLNLSIDVPKIDKGVDPSIIGGIDVGVKSPLVCAINNALSRYSISDNDLFHFNKKMFARRRILLRKNRHKRAGHGARNKLKPITIMTEKSKRFRKKLIERWACEIADFFIKNKVGTVQMENLESMKRKEDSYFNIRLRGFWPYAEMQNKIEFKLKQYGIVVRKVAPNNTSKTCSKCGHLNNYFNFEYRKKNKFPHFKCERCNFKENADYNAALNISNPKLKSTKGEP

SEQ ID NO: 671 - protein, 726 aa, synthetic construct
SEVEFSHEYWMRHALTLAKRARDEREVPVGAVLVLNNRVIGEGWNRAIGLHDPTAHAEIMALRQGGLVLQNYRLVDATLYVTFEPCTMCAGAMIHSRIGRVVFGVRNSKRGAAGSLMNVLNYPGMNHRVEITEGILADECAALICDYYRMPRQVFNARKKAQSSINSGGSSDGGSGSETPGTSESATPESSGGSSGGSAKNTITKTLKLRIVRPYNSAEVEKIVADEKNNREKIALEKNKDKVKEACSEHLKVAAYCTTQVERNACLFCKARRLDDKFYQKLRGQFPDAVFWQEIGEIFRQLQKQAAETYNQSLIELYYEIFIKGKGIANASNVEHYLSDVCYTRAAELFKNAAIASGLRNKIKSNFRLKELRNMKSGLPTTKSDNFPIPLVKQKGGQYTGFEISNHNGDFIIKIPFGRWQAKKEIDKYRPWEKFDFEQVRKSPKPISLLLSTQRRKRNRGWSKDEGTEAEIRKVMNGDYQTSYIEVKRGSKIGEKSAWMLSLSIDVPKIDKGVDPSIVGGIDVGVKSPLVCAINNALSRYSISDNDLFRFNKKMFARRRILLKKNRHKRAGHGAKNKLKPISILTGKSERFRKKLIERWACEIADFFIKNKVGTVQMENLESMKRREDSYFNIRLRGFWPYAEMQNRIEFKLKQYGIEIRKVAPNNTSKTCSKCGHLNNYFNFEYRKKNKFPHFKCEKCNFKENADYNAALNISNPKLKSTKEEP

SEQ ID NO: 672 - protein, 726 aa, synthetic construct
SEVEFSHEYWMRHALTLAKRARDEREVPVGAVLVLNNRVIGEGWNRAIGLHDPTAHAEIMALRQGGLVMQNYRLIDATLYVTFEPCVMCAGAMIHSRIGRVVFGVRNSKHGAAGSLVNVLNYPGMNHRVEITEGILADECAALLCDFYRMPRQVFNARKKAQSSINSGGSSGGSSGSETPGTSESATQESSGGGSSGPARNTITKTLRLRIVRPYNSAEVEKIVADEKNNREKIALEKNKDKVREACSKHLKVASYCTTQVERNACPFCKARKLDDKFYQKLRGQFPDAVFWQELGEILRQLQKQAAEIYNQSLIELYYEIFIKGKGAANASSVEHYLSDVCYTRAAGLFKNAAIASGLRGKVKSNFRLKELKNMKSGLPTTKSDNFPIPLVKQKGGQYTGFEISNHNDDFIIKIPFGRWQVKKEIDKYRPWEKFDFEQVRKSPKPISLLLSTQRRKRNKGWSKDEGTEAEIRKVMNGDYQTSYIEVKRGNKTGEKSAWMLNLSIDVPKIDKGVDPSIIGGIDVGVKSPLVCAVNNAFSRYSISDNELFHFNKKMFARRRILLGKNRHKRAGHGVKNKLKPITILTEKSGRFRKKLIERWACEIADFFVKNKVGTVQMENLESMKRKEDSYFNIKLRGFWPYAEMQNKIEFKLKQYGIKVRRVAPNNTSKTCSKCGHLNNYFSFEYRKKNKFPHFKCEKCNFKENADYNAALNISNPKLKSAKEEP

SEQ ID NO: 673 - protein, 726 aa, synthetic construct
SEVEFSHEYWMRHALTLARRARDEREVPVGAVLVLNNRVIGEGWNRAIGLHDPTAHAEIMALRQGGLVMQNYRLVDATLYVTFEPCVLCAGAMVHSRIGRVVFGVRNSKRGAAGSLMNVLNYPGMNHRVEITEGILADECAALLCDFYRMPRQVFNARKKARSNINSGGSSGGSSGSETPGASESATPKSSGGSSASSTKNTITKTLKLRIVRPYNSAEVEKIVADEKNNRERIALEKNKDKVKEACSQHLKMASYCTTQVERNACLFCKARKLDDKFYQKLRGQFPDAVFWQELGGIFRQLQRQAAEIYNQSLIELYYEIFIKGKGFANASSVEHYLSDVCYTRAAELFKNAAIASGLRGKVKGNFRLKELKNMKSGLPTTKSDNFPIPLVKQKGGQYTGFEISSHNDDFIIKIPFGRWQARKEIDKYRPWEKFDFEQVRKSPKPISLLLSTQRRKRNKGWGKDEGTEAEIRKVMNGDYQTSYIEVKRGSKIGEKSAWMLNLSIDVPKVDKGVDPNIIGGIDVGVRSPLVCAINNAFSRYSISDNDLFRFNKKMFARRRILLKKNRHKRAGHGAKNKLKPITILTKKSERFRKKLIERWVCEVADFFIKNKVGTVQMENLESMKRKEDSYFNIRLRGFWPYAEMQNRIELKLKQYGIEIRRVAPNNTSRTCSKCGHLNNYFNFEYRKKNKFPHFKCEKCNFREDADYNAALNISNPKLKSTKEEP

SEQ ID NO: 674 - protein, 726 aa, synthetic construct
SEVEFSHEYWMRHALTLAKRARDEREVPVGAILVLNNRVIGEGWNRAIGLHDPTAHAEIMALRQGGLVMQNYRLIDATLYVTFEPCVMCAGAMIHSRIGRVVFGVRNNKHGAAGSLVNVLNYPGMNHRVEITEGILADECAALLCDFYRMPRQVFNARKKAQSSINPGGSSGSSSGSETPGTSENATPESSGGSSGSSAKNTITKTLKLRIVRPYNSAEVEKIVADEKNNREKIALERNKDKVKEACSEHLKVAAYCTTQVERNACLFCKARKLDDRFYQKLRGQFPDAVFWQETGEIFRQLQRQAAEIYNQSLIELYYEIFIKGKGFANASSVEHYLSDVCYARAAELFKNAAIASGLRGKVKSNFRLKELKNMKSGLPTTKSDNFPIPLVKQKGGQYTGFEISSHNDDFIIKIPFGRWQVKKEIDKYRPWEKFDFEQVRKSPKPISLLLSTQRRKRNKGWSKDEGTEAEIRKVMNGDYQTSYIEVKRGSKIGEKSAWMLNLSIDVPKIDKGVDPSIIGGIDVGVKSPLVCAINNAFSRYSISDNDLFHFNKKMFARRRILLKKNRHKRAGHGAKNKLKPISILTEKSKRFRKKLIERWACEIADFFIKNKVGTVQMENLESMKRKEDSYFNIRLRGFWPYAEMQNKIEFKLKQYGIEIRKVAPNNTSKTCSKCGHLNNYFNFEYRKMNKFPHFKCEKCNFKENADYNAALNISNPKLKSTKEEP

SEQ ID NO: 675 - protein, 726 aa, synthetic construct
SEVEFSHEYWMRHALSLAKRARDEREVPVGAVLVLNNRIIGEGWNRAIGLHDPTAHAEIMALRQGGLVMQNYRLTDATLYVTFEPCVMCAGAMVHSRIGRVVFGVRNSKRGAAGSLMNVLNYPGANHCVEITEGILADECAALLCDYYRMPRQVFNARKKAQSGINSGGSSDGGSGSETPGTSESATPESSGGSSGGSAKNTITKTLKLRIVRPYNSAEVEKIVADEKNNREKIALEKNKGKVKEACSKHLKVAAYCTTQVERNACLFCKARKLDDKFYQKLRGQFPDAVFWQEVGEIFRQLQKQAAEIYNQSLIELYYEIFIKGKGFANASSVEHYLSDVCYTRAAELFKNAAIASGLRGKVKSNFRLKELKNMKSGLPTTKSDNFPIPLVKQKGGQYTGFEISNRNSDFIIKIPFGRWQVKKEINKYRPWEKFDFEQVRKSPKPISLLLSTQRRKRNKGWSKDEGTEAEIRKVMNGDYQTSYIEVKRGSRIGEKSAWMLSLSIDVPKIDRGVDPSIIGGIDVGVKSPLVCAINNALSRYSISDNDLFHFNKKMFARRRILLKKNRHRRAGHGARNKLKPITVLTEKSKRFRKKLIERWACEIADFFIKNKVGTVQMENLESMKRKEDSYFNIRLRGFWPYAEMQNKIEFKLKQYGIVVRKVAPNNTSKTCSKCGHLNNYFNFEYRKKNKFPHFKCEKCNFKENADYNAALNISNPKLKSTKGEP

SEQ ID NO: 676 - protein, 726 aa, synthetic construct
SEVEFSHEYWMRRALTLAKRARDEREVPVGAVLVLNNRVIGEGWNRAIGLHDPTAHAEIMALRQGGLVMQNYRLIDATLYVTFEPCVMCAGAMIHSRVGRVVFGVRNSKHGAAGSLMNVLNYPGMNHRVEITEGILADECAALLCEFYRMPRRVFNARKKAQSSIDPGGPSGGSSGSETPGSSESTTPESSGSGSSGSAKNTITKTLQLRIVRPYNSAEVEKIVADEKNNREKIALEKNKDKVKGACSKHLKVASYCTTQVERNACPFCKARKLDDKFYQKLRGQFPDAVFWQELGEILRQLQKQAAEIYNQSLIELYYEIFIKGKGITNASRVEHYLSDVCYTRAAELFKNAAIASGLRSKVRSNFRLKELKNMKSGLPTTKSDNFPIPLVKQKGGQYTGFEISSHNSDFIIKIPFGRWQVKKEIDKYRPWEKFDFEQVRKSPKPISLLLSTQRRRRNKGWSKDEGTEAEIRKVMNGDYQISYIEVRRGRKIGEKSAWMLNLSIDVPKIDKGVDPSIVGGIDVGVKSPLVCAINNALGRYSISDNDLFHFNKKMFARRRILLKKNGHKRAGHGTKNKLKPISILTEKSKRFRKKLIERWACEIADFFIKNKVGTVQMENLESMKRKEDSYFNIRLRGFWPYAEMQNKIEFKLKQYGIKIRKVAPNNTSKTCSKCGHLNNYFSFEYRKKNKFPHFKCEKCNFKEDADYNAALNISNPKLKSTKEEP

SEQ ID NO: 677 - protein, 726 aa, synthetic construct
SEVEFSHEYWMRHALTLAKRARDEREVPVGAVLVLNNRVIGEGWNRAIGLHDPTAHAEIMALRQGGLVMQNYRLTDATLYVTFEPCVMCAGAMIHSRIGRVVFGVRNSKRGAAGSLMNVLNYPGMNHCVEITEGILVDECAALLCDFYRMPRQVLNAQKKAQSSISPGGSSGGSSGSETPGASGSVTPKSSGGSSAGSAKNTITKTLQLRIVRPYNSAEVEKIVADEKNNREKIALEKNRDKVKEACSEHLKVAAYCTTQVERSACLFCKARKLDDKFYQKLRGQFPDAVFWQEIGEIFRQLQKQAAEIYNQSLIELYYEIFIKGKGFANASSVEHYLSDVCYTRAAELFKNAAIASGLRGKVKSNFRLKELKNMKSGLPTTKSDNFPIPLVKQKGGQYTGFEVGSHNSDFIIKIPFGRWQVKEEIDKYRPWEKFDFEQVRKSPKPISLLLSTQRRKKNKGWSKDEGTEAEIRRVMNGDYQTSYIEVKRGSKIGEKSAWMLNLSIDVPKIDKGVDPSIIGGIDVGVKSPLVCAINNSLSRYSICDNDLFRFNKKMFARRRILLKKNRHKRAGHGAKNKLKPITILTKKSERFRKKLIERWACEIANFFIKNKVGTVQMENLESMKRREDSYFNIRLRGFWPYAEMQNKIEFKLKQYGIEIRKVAPNNTSKTCSKCGHLNNYFNFEFRKKNKFPHFRCEKCNFKENADYNAALNISNPKLKSTKEEP

SEQ ID NO: 678 - protein, 726 aa, synthetic construct
SEVEFSHEYWMRHALTLAKRARDEREVPVGAILVLNNRVIGVGWNRAIGLHDPTAHAEIMALRQGGLVLQNYRLIDATLYVTFEPCVMCAGAMIHSRIGRVVFGVRNSKHGAAGSLVNVLNYPGMNHRVEITEGILADECAALLCDFYRMPRQVFNARKKAQSSINSGGSSGGSSGSETPGTSESATPESSGGSSGSSAKNTITKTLKLRIVRPYNSAEVEKIVADEKNNREKIALEKNKDKVKEACSKHLKVAAYCTTQVERNACLFCKARRLDDKFYQKLRGQFPDAVFWQEIGEIFRQLQKQAAEVYNQSLVELYYEILIKGKGIANASSVEHYLSNVCYTRAAELFKNAAIASGLRNKIKSNFRLKELRNMKSGLPTTKSDNFPIPLVRQKGGQYTGFEISNHDGDFIIKIPFGRWQVKKEINKHRPWEKFDFEQVRKSPKPISLLLSTQRRKRNKGWSKDEGTEAEIRKVMNGDYQTSYIEVKRGSKIGEKSAWMLNLSIDVPKIDKGVDPGIIGGIDVGVKSPLVCAINNALSRYSISDNDLFHFNKKMFARRRILLRKNRHKRAGHGAKNKLKPITMMTEKSKRFRKKLIERWACEIADFFIKNKVGTVQMENLESMKRKEDSYFNIRLRGFWPYAEMQNKIEFKLKQYGIVVRKVAPNNTSKTCSKCGHLNNYFDFEYRKKNKFPHFKCEKCNFKEDADYNAALNISNPKLKSSKGEP

SEQ ID NO: 679 - protein, 726 aa, synthetic construct
SEVEFSHEYWMRHALTLAKRARDEREVPVGAVLVLNNRVIGEGWNRAIGLHDPTAHAEIMALRQGGLVMQNYRLIDATLYVTFEPCVMCAGAMIHSRIGRVVFGVRNSKHGAAGSLVNVLNYPGMNHRVEITEGILADECAALLCDFYRMPRQVFNARKKAQSSINSGGSSGGSSGSERPGTSESATPESSGGSSGGSAKNTITKTLKLRIVRPYNSAEVEKIVADEKNYREKIALERNKDKVKEACSEHLKVAAYCTTQVERSACLFCKARKLDDKFYQKLRGQFPDAVFWQEIGEIFRQLQKQAAEIYNQSLIELYYEIFIKGKGFANASSVEHYLSDVCYTRAAELFKNAAIASGLRSKVRSNFRLKELKNMKSGLPTTKSDNFPIPLVKQKGGQYTGFEISSHNSDFIIKIPFGRWQVKEEIDKYRPWEKFDFEQVRKSPKPISLLLSTQRRKKNKGWSKDEGTEAEIRRVMNGDYQTSYIEVKRGSKIGEKSAWMLNLSIDVPKIDKGVDPSIIGGIDVGVKSPLVCAINNAFSRYSISDNDLFHFNKKMFARRRILLKKNRHKRAGHGAKNKLKPISILTEKSKRFRKKLIERWACEIADFFIKNKVGTVQMENLESMKRKEDSYFNIRLRGFWPYAEMQNKIEFKLKQYGIEIRKVAPNNTSKTCSKCGHLNNYFNFEYRKKNKFPHFKCEKCNFKENADYNAALNISNPKLKSTKEEL

SEQ ID NO: 680 - protein, 726 aa, synthetic construct
SEVEFSHEYWMRHALTLAKRARDEREVPVGAVLVLNNRVIGEGWNRAIGLHDPTAHAEIMALRQGGLVMQNYRLTDATLYVTFEPCVMCAGAMIHSRIGRVVFGVRNSKRGAAGSLMNVLNYPGMNHCVEITEGILVDECAALLCDFYRMPRQVLNAQKKAQSSISSGGSSGGSSGSETPGVSESATPKSSGGSSAGSTKNTITKALKLRIVRPYNSAEVEKIVADEKNNREKIALEKNKDKVKEACSEHLKVVAYCTTQVERNACLFCKARKLDDKFYQKLRGQFPDAVFWQETGEIFRQLQRQAAEIYNQSLIELYYEIFIKGKGFANASSVEHYLSDVCYTRAAELFKNAAIASGLRGKVKSNFRLKELKNMKSGLPTTKSDNFPIPLVKQKGGQYTGFEISSHNDDFIIKIPFGRWQVKKEIDKYRPWEKFDFEQVRKSPKPISLLLSTQRRKRNKGWSKDEGTEAEIRKVMNGDYQTSYIEVKRGSKTGEKSAWMLNLSIDVPKIDKGVDPSIIGGIDVGVKSPLVCAINNAFSRYSISDNDLFRFNKKMFARRRILLKKNRHKRAGHGAKNKLKPISILTEKSKRFRKKLIERWACEIADFFIKNKVGTVQMEDLESMKRKEDSYFNIRLRGFWPYAEMQNKIEFKLKQYGIEIRKVAPNNTSKTCSKCGHLNNYFNFEYRKKNKFPHFKCEKCNFKENADYNAALNISNPKLKSTKEEP

SEQ ID NO: 681 - protein, 726 aa, synthetic construct
SEVEFSHEYWMRHALTLAKRARDEREVPVGAVLVLNNRVIGEGWNRTTGLHDPTAHAEIMALRQGGLVMRNYRLTDATLYVTFEPCVMCAGAMIHSRIGRVVFGVRNSKRGAAGSLMNVLNYPGMNHRVEITEGILADECAALLCDFYRMPRQVFNARKKAQSSINPGGPSGGSSGSETPGTSESATPESSGGGSSGSAKSTITKTLQLRIVRPYNSAEVEKIVAEEKNNREKIALEKNKDKVKEACSKHLKVAAYCTTQVERNACLFCKARKLDDKFYQKLRGQFPDAVFWQEIGEIFRQLQKQAAEIYNQSLIELYYEIFIKGKGFANASSVEHYLSDVCYTRAAGLFKNAAIASGLRGKVKSNFRLKELKNAKSGLPTTKSDNFPIPLVKQKGGQYTGFEISNHDGDFIIKIPFGRWQVKKEIDKYRPWEKFDFEQVRKSPKPISLLLSTQRRKRNKSWSKDEGTEAEIRKVMNGDYQTSYIEVKRGSKIGEKSAWMLNLSIDVPKIDKGVDPSIVGGIDVGVKSPLVCAINNAFSRYSISDNDLFHFNKKMFARRRILLKKNRHKRAGHGAKNKLKPISILTEKSKRFRKKLIERWACEIADFFIKNKVGTVQMENLESMKGKEDSYFNIRLRGFWPYAEMQNKIEFKLKQYGIEIRKVAPNNTSKTCSRCGHLNNYFNFEYRKMNKFPHFKCEKCNFKENADYNAALNISNPKLKSTKEEP

SEQ ID NO: 682 - protein, 726 aa, synthetic construct
SEDEFSHEYWMRHALTLAKRARDGREVPVGAVLVLNNRVIGEGWNRAIGLHDPTAHAEIMALRQGGLVMQNYRLIDATLYVTFEPCVMCAGAMIHSRIGRVVFGVRNSKHGAAGSLVNVLNYPGMNHRVEITEGILADECAALLCDFYRMPRQVFNARKKAQPSINPGGSSGGSSGSETPGTSESATPESSGGSSGGSAKNTITKTLQLRIVRPYNSAEVEKIVADEKNNRERIALEKNKDKVKEACSKHLKVAAYCTTQVERNACLFCKARKLDDKFYQKLRGQFPDAVFWQELGGIFRQLQKQAAEIYNQSLIELYYEIFIKGKGITNASRVEHYLSDVCYTRAAELFKNAAIASGLRSKVRSNFRLKELKNMKSGLPTTKSDNFPIPLVKQKGGQYTGFEISSHNSDFIIKIPFGRWQEKEEIDKYRPWEKFDFEQVRRSPKPISLLLSTQRRKKNKGWSKDEGTEAEIRRVMNGDYQTSYIEVKRGSKIGEKSAWMLNLSIDVPKIDKGVDPSIIGGIDVGVKSPLVCAINNAFSRYSISDNDLFHFNKKMFARRRILLKKNRHKRAGHGAKNKLKPITILTEKSRRFRKKLIERWACEIADFFIKNKVGTVQMESLESMKRKEDSYFNIRLRGFWPYAEMQNKIEFKLKQYGIEIRKVAPNNTSKTCSKCGHLNNYFSFEYRKKNKFPHFKCEKCNFKENADYNAALNISNPKLKSTKEEP

SEQ ID NO: 683 - protein, 726 aa, synthetic construct
SEVEFSHEYWMRHALTLAKRARDEREVPVGAILVLNNRVIGEGWNRAIGLHDPTAHAEIMALRQGGLAMQNYRLIDATLYVTFEPCVMCAGAMIHSRIGRVVFGVRNSKHGAAGSLMNVLNYPGMNHRVEITEGILADECAALLCDFYRMSHQVFNARKKAQSSINPGGPSGGSSGSETPDTSESATPESSGGNSGGSAKNTITKTLKLRIVRPYNSAEVEKIVADEKNNRERIALEKNKDKVKEACSKHLKVAAYCTTQVERNACLFCRARKLDDKFYQKLRGQFPDAVFWQEIGEIFRQLQKQAAEIYNQSLIELYYEIFIKGKGFANASSVEHYLSDVCYTRAAELFKNAAIASGLRGKVKGNFRLKELKNMKSGLPTTKSDNFPIPLVKQKGGQYTGFEISSHNDDFIIKIPFGRWQAKKEIDRYRPWEKFDFEQVRKSPKPISLLLSTQRRKRNKGWSKDEGTEAEIRKVMNGDYQTSYIEVRRGSKIGEKSAWMLNLSIDVPKIDKGVDPSIIGGIDVGVKSPLVCAINNAFSRYSISDNDLFHFNKKMFARRRILLKKNRHRRAGHGAKNKLKPISILTEKSKRFRKKLIERWACEIADFFIKNKVGTVQMENLESMKRKEDSYFNIRLRGFWPYAEMQNKIEFKLKQYGIVVRKVAPNNTSKTCSKCGHLNNYFDFEYRKKNKFPHFKCEKCNFKEDADYNAALNISNPKLKSTKGEP

SEQ ID NO: 684 - protein, 726 aa, synthetic construct
SEDEFSHEYWMRHALTLAKRARDGREVPVGAVLVLNNRVIGEGWNRAIGLHDPTAHAEIMALRQGGLVMQNYRLIDATLYVTFEPCVMCAGAMVHSRIGRVVFGVRNSKRGAAGSLMNVLNYPGMGHRVEITEGILADECAALLCDFYCMPRQVFNAQKRAQFSINSGGSSGGSSGSETPGSSESATPESSGGGSSGSAKNTITKALQLRIVRPYNSAEVEKIVADEKNNREKIALEKNKDKVKEACSKHLKVASYCTTQVERNACPFCKARKLDDKFYQKLRGQFPDAVFWQELGEILRQLQKQAAEIYNQSLIELYYEIFIKGRGFANAGSVEHYLSDVCYTRAAELFKNAAIASGLRGKVKSNFRLKELKNMKSGLPTTKSDNFPIPLVKQKGGQYTGFEISSHNDDFIIKIPFGRWQVKKEIDKYRPWEKFDFEQVRKSPKPISLLLSTQRRKRNKGWSKDEGTEAEIRKVMNGDYQTSYIEVKRGSKTGEKSAWMLNLSIDVPKIDKGVDPSIIGGIDVGVKSPLVCAINNAFSRYSISDNDLFRFNKKMFARRRILLKKNRHKRAGHGAKNKLKPISILTGKSERFRKKLIERWACEIADFFIKNKVGTVQMENLESMKRKEDSYFNIRLRGFWPYAEMQNKIEFKLKQYGIEIRRVAPNNTSKTCSKCGHLNNYFNFEYRKKNKFPHFKCEKCNFKENADYNAALNISNPELKSTKEEP

SEQ ID NO: 685 - protein, 726 aa, synthetic construct
SEVEFSHEYWMRHALTLAKRARDEREVPVGAILVLNNRVIGEGWNRAIGLHDPTAHAEIMALRQGGLVMQNYRLTDATLYVTFEPCVMCAGAMIHSRIGRVVFGVRNSKRGAAGSLMNVLNYPGMNHCVEITEGILVDECAALLCDFYRMPRQVLNAQKKAQSSINSGGPSGGSSGSEAPGTSESATPESSGGGSSGSAKNTITKTLQLRIVRPYNSAEVEKIVADEKNNREKIALEKNKDRVKEACSKHLKVASYCTTQVERNACPFCKARRLDDKFYQKLRGQFPDAMFWQELGEILRQLQKQAAEIYNQSLIELYYEIFIKGRGFANAGSVEHYLSDVCYTRAAELFKNAAIASGLRGKVKSNFRLKELKNMKSGLPTTKSDNFPIPLVKQKGGQYTGFEISSHNDDFIIKIPFGRWQVKKEIDKYRPWEKFDFEQVRKSPKPISLLLSTQRRKRNKGWSKDEGTEAEIRKVMNGDYQTSYIEVKRGSKIGEKSAWMLNLSIDVPKIDKGVDPSIIGGIDVGVKSPLVCAINNAFGRYSISDNDLFHFNKKMFARRRILLKRNRHKRAGHGAKNKLKPITILTEKSKRFRRKLIERWACEIADFFIKNKVGTVQMENLEGMKRKEDSYFNIRLRGFWPYAEMQDKIEFKLKQYGIVVRKVAPNNTSKTCSKCGHLNNYFNFEYRKKNKFPHFKCEKCNFKENADYNAALNISDPKLKSTKKEP

SEQ ID NO: 686 - protein, 726 aa, synthetic construct
SEVEFSHEYWMRRALTLAKRARDEREVPVGAVLVLNNRVIGVGWNRAVGLHDPTAHAEIMALRQGGLVMQNYRLVEATLYVTFEPCIMCAGAMIHSRIGRVVFGVRNSKRGAAGSLMNVLNHPGMNHRVEITEGILADECAALLCDYYRMPRQVFNARKKAQPSINSGGSSDGGSGSETPGTSESATPESSGGSSGGSAKNTITKTLKLRIVRPYNSAEVEKIVADEKNYREKIALEKNKDKVQEACSKHLKVASYCTTQVERNACLFCKARKLDDKFYQKLRGQFPDAVFWQELGEIFRQLQKQAAEIYNQSLIELYYKIFIKGKGLANASNVEHYLSDVCYTRAAELFKNAAIASGLRGKVKSNFKLKELKSMKSGLPSTKSDNFPIPLVKQKGGQYTGFEISSHNDDFIIKIPFGRWQVKEEIDKYRPWEKFDFEQVRKSPKPISLLLSTQRRKRNKGWSKDEGTEAEIRKVMNGDYQTSYIEVKRGSKIGEKSAWMLNLSIDVPKIDKGVDPSIVGGIDVGVKSPLVCAIANALSRYSISDNDLFHFNKKMFARRRILLKKNRHRRAGHGAKNKLKPISILTEKSKRFRKKLIERWASEIADFFIKNKVGTVQMENLESMKRKEDSYFNIRLRGFWPYAEMQSKIEFKLKQYGIEVRKVAPNNTSKTCSKCGHLNNYFNFEYRKKNKFPHFKCEKCNFKENADYNAALNISNPKLKSTKEEP

SEQ ID NO: 687 - protein, 726 aa, synthetic construct
SEVEFSHEYWMRHALTLAKRARDEREVPVGAVLVLNNRVIGEGWNRAIGLHDPTAHAEIMALRQGGLVMQNYRLIDATLYVTFEPCVMCAGAMVHSRIGRVVFGVRNSKRGAAGSLMNVLDYPGMGHRVEITEGILADECAALLCDFYRMPCQVFNAQKRAQSSINSGGSSGGSSGSETPGASGSVTPKSSVGSSAGSTKNTITKTLQLRIVRPYNSAEVEKIVADEKNNREKIALEKNKDKVKEACSKHLKVAPYCTTQVERNACPFCKARKLDDKFYQKLRGQFPDAVFWQELGEILRQLQKQAAEIYNQSLIELYYEIFIKGRGFANAGSVEHYLSDVCYTRAAELFKNAAIASGLRGKVKSNFRLKELKNMKSGLPTTKSDNFPIPLVKQKGGQYTGFEISSHNDDFIIKIPFGRWQVKEEIDKYRPWEKFDFEQVRKNPKPISLLLSTQRRRGNKGWSKDEGTEAEIRKVMNGDYQTSYIEVKRGSKIGEKSAWMLNLSIDVPKIDKGVDPSIIGGIDVGVKSPLVCAINNAFSRYSISDNDLFRFNKKVFARRRILLKKNRHKRAGHGTKNKLKPITILTEKSGRFRKKLIERWACEIANFFVKNKVGTVQMEDLESMKRKEDSYFNIRLRGFWPYAEMQNKIEFKLKQYGIKIRKVAPNNTSKTCSKCGHLNNYFNFEYRKKNKFPHFKCEKCNFKEDADYNAALNISNPKLKSTKEEP

SEQ ID NO: 688 - protein, 726 aa, synthetic construct
SEVEFSHEYWMRHALALAKRARDEREVPVGAVLVLNNRVIGEGWNRAIGLHDPTAHAEIMALRQGGLVMQNYRLVDATLYVTFEPCVLCAGAMVHSRIGRVVFGVRNSKRGAAGSLMNVLNYPGMNHRVEITEGILADECAALLCDFYRMPRQVFNAQKKAQSSINPGGPSGGSSGSETSDTSESATPESSGGNSGGSAKNTITKTLKLRIVRPYNSAEVEKIVADEKNNREKIALEKNKDKVKEACSEHLKVAAYCTTQVERNACLFCKARKLDDKFYQKLRGQFPDAVFWQELGEIFRQLQKQTAEIYNQSLIELYYEIFIKGKGFANASSVEHYLSDVCYTRAAELFKNAAIASGLRGKVKSNFRLKELKNMKSGLPTTKSDNFPIPLVKQKGGQYTGFEISSHNDDFIIKIPFGRWQMKKEIDRYRPWEKFDFEQVRKSPKPISLLLSTQRRKRNKGWSKDEGTEAEIRKVMNGDYQTSYIEVRRGSKIGERSAWMLNLSIDVPKIDKGVNPSIIGGIDVGVKSPLVCAINNAFSRYSISDNDLFRFNKKMFARRRILLGKNRHKRAGHGVKNKLKPITILTEKSGRFRKKLIERWACEIADFFIKNKVGTVQMENLESMKRKEDSYFNIRLRGFWPYAEMQNKIELKLKQYGIKIRKVAPNNTSKTCSKCGHLNDYFDFEYRKKNKFPHFKCEKCNFKENADYNAALNISNPKLKSTKEEP

SEQ ID NO: 689 - protein, 726 aa, synthetic construct
SEVEFSHEYWMRHALSLAKRARDEREVPVGAVLVLNNRIIGEGWNRAIGLHDPTAHAEIMALRQGGLVMQNYRLTDATLYVTFEPCVMCAGAMVHSRIGRVVFGVRNSKRGAAGSLMNVLNYPGVNHCVEITEGILVDECAALLCDFYRMPRQVLNAQKKAQSSISSGGSSGGCSGGEMPGASESVTPKSSGGSSAGSTKNTITKTLKLRIVRPYNSAEVEKIVADEKNSREKIALERNKDKVKEACSEHLKVAAYCTTQVERNACLFCKARKLDDRFYQKLRGQFPDAVFWQETGEIFRQLQRQAAEIYNQSLIELYYEIFIKGKGFANASSVEHYLSDVCYTRAAELFKNAAIASGLRGKVKSNFRLKELKNMKSGLPTTKSDNFPIPLVKQKGGQYTGFEISSHNDDFIIKIPFGRWQVKKEIDKYRPWEKFDFEQVRKSPKPISLLLSTQRRKRNKGWSKDEGTEAEIRKVMNGDYQTSYIEVKRGSKIGEKSAWMLNLSIDVPKIDKGVDPSIIGGIDVGVKSPLVCAINNALSRYSISDNDLFHFNKKMFARRRILLKKNGHKRAGHGAKNKLKPITIMTEKSKRFRKKLIERWACEIADFFIKNKVGTVQMENLESMKRKEDSYFNIRLRGFWPYAEMQNKIEFKLKQYGIVVRKVAPNNTSKTCSQCGHLNNYFSFEYRKKNKFPHFKCEKCNFKEDADYNAALNISNPKLKSTKEEP

SEQ ID NO: 690 - protein, 726 aa, synthetic construct
SEVEFSHEYWMRHALTLAKRARDEREVPVGAVLVLNNRVIGEGWNRAIGLHDPTAHAEIMALRQGGLVMQNYRLTDATLYVTFEPCVMCAGAMIHSRIGRVVFGVRNSKRGAAGSLMNVLNYPGMNHCVEITEGILVDECAALLCDFYRMPRQVLNTQKKARSNINSGGSSGGSSGSETLGTSESATPESSGGSSGGSAKNTITKTLKLRIVRPYNSAEVEKIVADEKNNREKIALEKNKDKVKEACSKHLKVASYCTTQVERNACLFCKARKLDDKFYQKLRGQFPDAVFWQELGEIFRQLQKQAAEIYNQSLIELYYEIFIKGKGLANASSVEHYLSDVCYTRAAELFKNAAIASGLRGKVKSNFRLKELKNMKSGLPTTKSDNFPIPLVKQKGGQYTGFEISSHNDDFIIKIPFGRWQVKEEIDKYRPWEKFDFEQVRKGPKPISLLLSTQRRKRNKGWSKDEGTEAEIRKVMNGDYQTSYIEVQRGSKIGEKSAWMLNLSIDVPKIDKGVDPSIIGGIDVGVKSPLVCAINNAFSRYSISDNDLFHFNKKMFARRRILLKKNGHKRAGHGAKNKLKPITIMTEKSKRFRKKLIERWACEIADFFIKNKVGTVQMENLESMKRKEDSYFNIRLRGFWPYAEMQNKIEFKLKQYGIVVRKVAPNNTSKTCSQCGHLNNYFNFEYRKKNKFPYFKCEKCNFKENADYNAALNISNPKLKSTKEEP

SEQ ID NO: 691 - protein, 726 aa, synthetic construct
SEVEFSHEYWMRHALTLAKRARDEREVPVGAVLVLNNRVIGEGWNRTTGLHDPTAHAEIMALRQGGLVMQNHRLVDATLYVTFEPCVMCAGAMIHSRIGRVVFGVRNSKRGAAGSLTNVLDYPGMNHRVEITEGILVDECAALLCDFYRMPRQVFNAQKKAQSTINSGGSSGGSSGSETPGTSESPTPESSGGSPGGSAKNTITKTLRLRIVRPFNSAEVEKIVADEKNNREKIALEKNKDKVKEACSKHLKMASYCTTQVERNACLFCKARKLDDKFYQKLRGQFPDAVFWQELGGIFRQLQKQAAEIYNQSLIELYYEIFIKGKGITNAGRVEHYLSDVCYTRAAELFKNAAIASGLRSKVRSNFRLKELKSMKSGLPTTKSDNFPIPLVKQKGGQYTGFEISSHNSDFIIKIPFGRWQVKEEIDKYRPWEKFDFEQVRKSPKPISLLLSTQRRKKNKGWSKDEGTEAEIRRVMNGDYQTSYIEVKRGSKIGEKSAWMLNLSIDVPKIDKGVDPSIIGGIDVGVKSPLVCAINNSSSRYSICDNDLFRFNKKMFARRRILLKKNRHKRAGHGAKNKLKPITILTKKSERFRKKLIERWVCEVADFFIKNKVGTVQMENLESMKRKEDSYFNIRLRGFWPYAEMQNKIEFKLKQYGIEIRRVAPNNTSRTCSKCGHLNSYFNFEYRRKYKFPHFKCEKCNFKEDADYNAALNISNPKLKSTKEEP

SEQ ID NO: 692 - protein, 726 aa, synthetic construct
SEVEFSHEYWMRHALTLAKRARDEREVPVGAVLVLNNRIIGEGWNRAIGLHDPTAHAEIMALRQGGLVMQNYRLIDATLYVTFEPCVMCAGAMIHSRIGRVVFGVRNSKHGAAGSLVNVLNYPGMNHRVEITEGILADECAALLCDFYRMPRRVFNARMKAQSSISPGGSSGGSSGSETPGTSESATPESSGGSSGGSAKNTITKTLQLRIVRPYNSAEVEKIVADEKNNREKIALEKNKDKVREACSKHLKVASYCTTQVERNACPFCKARKLDDKFYQKLRGQFPDAVFWQELGEILRQLQKQAAEIYNQSLIELYYEVFIKGRGFANASSVEHYLSDVCYTRAAELFKNAAIASGLRGKVKSNFRLKELKNMKSGLPTTKSDNFPIPLVKQKGGQYTGFEISSHNDDFIIKIPFGRWQVKKEIDKYRPWEKFDFEQVRKSPKPISLLLSTQRRKRNKGWSKDEGTEAEIRKVMNGDYQTSYIEVKRGSKTGEKSAWMLNLSIDVPKIDKGVDPSIIGGIDVGVKSPLVCAINNAFSRYSISDNDLFRFNKKMFARRRILLKKNRHKRAGHGAKNKLKPFTILTEKSGRFRKKLIERWACEIADFFVKNKVGTVQMENLESMKRKEDSYFNIRLRGFWPYAEMQNRIEFKLKQYGIKVRKVAPNNTSKTCSKCGHLNSYFSFEYRKKNKFPHFKCEKCNFKENADYNAALNISNPKMKSTKEEP

SEQ ID NO: 693 - protein, 726 aa, synthetic construct
SEVEFSHEYWMRHALTLAKRARDEREVPVGAVLVLNNRVIGEGWNRTTGLHDPTAHAEIMALRQGGLVMQNHRLVDATLYVTFEPCVLCAGAMVHSRIGRVVFGVRNSKRGAAGSLMNVLNYPGMNHRVEITEGILADECAALLCDFYRMPRQVFNARKKAQSSINSGGSSDGGSGNETPGTSESATPESSGGSSGGSAKNTITKTLKLRIVRPYNSAEVEKIVADEKNNRVKIALEKNKDKVKEACSEHLKVAAYCTTQVERSACLFCKARKLDDKFYQKLRGQFPDAVFWQEIGEIFRQLQKQAAEIYNQSLIELYYEIFIKGKGFANASSVEHYLSDVCYTRAAELFKNAAIASGLRGKVKSNFRLKELKNMRSGLPTAKSDNFPIPLVKQKGGQYTGFEVSSHNDDFIIKIPFGRWQVKKEIDKYRPWEKFDFEQVRKSPKPISLLLSTRRRKGNKGWSKDEGTEAEIRKVMNGDYQTSYIEVKRGSKIGEKSAWMLSLSIDVPKIDKGVDPRIIGGIDVGVKSPLVCAINNVLSRYSISDNDLFHFNKKMFARRRILLKKNGHKRAGHGAKNKLKPITIMTEKSKRFRKKLIERWACEIADFFIKNKVGTVQMENLESMKRKEDSYFNIRLRGFWPYAEMQNKIEFKLKQYGIVVRKVAPNNTSKTCSQCGHLNNYFNFEYRKKNKFPYFKCEKCNFKENADYNAALNISNPQLKSTKGEP

SEQ ID NO: 694 - protein, 726 aa, synthetic construct
SEVEFSHEYWMRHALTLAKRARDEREVPVGAVLVLNNRVIGEGWNRAIGLHDPTAHAEIMALRQGGLVMQNHRLVDATLYVTFEPCVMCAGAMIHSRIGRVVFGVRNSKRGAAGSLTNVLNYPGMNHRVEITEGILVDECAALLCDFYRMPRQVFNAQKRAQSTINTGGSSGGSSGSETPGTSESPTPESSGGSPGGSAKNTITKTLKLRIVRPYNSAEVEKIVADEKNNREKIALEKNKDKVKEACSEHLKVAAYCTTQVERSACLFCKARKLDDKFYQKLRGQFPDAVFWQEVGEIFRQLQKQAAEIYNQSLIELYYEIFIKGKGFANASSVEHYLSDVCYTRAAELFKNAAIASGLRGKVKSNFRLKELKNMKSGLPTTKSDNFPIPLVKQKGGQYTGFEISSHNDDFIIKIPFGRWQVKKEIDKYRPWEKFDFEQVRKSPKPISLLLSTQRRKRNKGWSKDEGTEAEIRKVMNGDYRTSYIEVKRGSKTGEKSAWMLNLSIDVPKIDKGVDPSIIGGIDVGVKSPLVCAINNAFSRYSISDNDLFRFNKKMFARRRILLRKNRHKRAGHGAKNKLKPISILTGKSERFRKKLIERWACEIADFFIKNKVGTVQMENLESMKRKEDSYFNIRLRGFWPYAEMQNKIEFKLKQYGIEIRKVAPNNTSKTCSKCGHLNNYFNFEYRKKNKFPHFKCEKCNFKENADYNAALNISNPKLKSTKEEP

SEQ ID NO: 695 - protein, 726 aa, synthetic construct
SEVEFSHEYWMRHALSLAKRARDEREVPVGAVLVLNNRIIGEGWNRAIGLHDPTAHAEIMALRQGGLVMQNYRLINATLYVTFEPCVMCAGAMIHSRIGRVVFGVRNSKHGAAGSLMNVLNYPGMNHRVEITEGILADECAALLCDFYRMPRQVFSARKKAQSSINSGDSSGGNSGNKTPGTSESATPESSGGSSGGSAKNTITKTLKLRIVRPYNSAEVEKIVADEKNNREKIALEKNKDKVKEACSKHLKVAAYCTTQVERNACQFCKARKLDDKFYQKLRGQFPDAVFWQEIGEIFRQLQKQAAEIYNQSLIELYYEIFIRGKGFANASSVEHYLSDVCYTRAAELFKNAAIASGLRGKVKSNFRLKELKNMKSGLPTTKSDNFPIPLVKQKGGQYTGFEISSHNDDFIIKIPFGRWQVKKEIDKYRPWEKFDFEQVRKSPKPISLLLSTQRRKRSKGWSKDEGTEAEIRKVMNGDYQTSYIEVKRGSKIGEKSAWMLNLSIDVPKIDKGVDPSIIGGIDVGVKSPLVCAINNAFSRYSVGDNDLFHYNKKMFARRRILLKKNRHKRAGHGAKNKLKPISILTEKSKRFRKKLIERWACEIADFFIKNKVGTVQIENLESMKRKEDSYFNIRLRGFWPYAEMQNKIEFKLKQYGIEIRKVAPNNTSKTCSKCGHLNSYFNFEYRKKNKFPHFKCEKCNFKEDADYNAALNISNPKLKSTKGEP

SEQ ID NO: 696 - protein, 726 aa, synthetic construct
SEVEFSHEYWMRHALTLAKRARDEREVPVGAILVLNNRVIGEGWNRAIGLHDPTAHAEIMALRQGGLVMQNYRLIDATLYVTFEPCVMCAGAMIHSRIGRVVFGVRNNKRGAAGSLMNVLNYPGMNHRVEITEGILAGECAALLCDFYRMPRQVLNAQKKTRSCINSGGSSGGSSGSETPGTSESATPESSGGSSGGSAKNTITKTLKLRIVRPYNSAEVEKIVADEKDNRERIALEKNKGKVKEACGKHLKVAAYCTTQVERNACLFCKARKLDDKFYQELRSQFPDAVFWQEIGEIFRQLQKQAAEIYNQSLIELYYEIFIKGKGFANASSVEHYLSDVCYTRAAELFKNAAIASGLRGKVKSSFRLKELKNMRSGLPTTKSDNFPIPLVKQKGGQYTGFEISSHNDDFIIKIPFGRWQVKKEIDKYRPWEKFDFEQVRKSPKPISLLLSTRRRKRNKGWSKDEGTEAEIRKVMNGDYQTSYIEVKRGSKIGEKSAWMLNLSIDVPKIDKGVDPSIIGGIDVGVKSPLVCAINNAFSRYSISDNELFHFNKKVFARRRILLKKNRHKRAGHGTKNKLKPITILTEKSGRFRKKLIERWACEIANFFIKNKVGTVQMENLESMKRKEDSYFNIRLRGFWPYAEMQNKIEFKLKQYGIKIRKVAPNNTSKTCSKCGHLNNYFSFEYRKKNKFPHFKCEKCNFKEDADYNAALNISNPKLKSTKEEP

SEQ ID NO: 697 - protein, 726 aa, synthetic construct
SEVEFSHEYWMRHALTLAKRARDEREVPVGAVLVLNNRVIGEGWNRAIGLHDPTAHAEIMALRQGGLVMQNYRLIDATLYVTFEPCVMCAGAMIHSRIGRVVFGVRNNKRGAAGSLMNVLNYPGMNHRVEITEGVLADECAALLCDFYCMPRQVLNARKKARSCINSGGSSGGSSGSETPGTSESATPESSGGSSGGSAKNTITKTLKLRIVRPYNSAEVEKIVADEKDNRERIALEKNKGKVKEACSKHLRVAAYCTTQVERNACLFCKARKLDDKFYQELRGQFPDAVFWQEIGEIFRQLQKQAAEIYNQSLIELYYEIFIKGKGFANASSVEHYLSDVCYTRAAELFKNAAIASGLRGKVKSNFRLKELKNMRSGLPTTKSDNFPIPLVKQKGGQYAGFEISSHNDDFIIKIPFGRWQVKKEIDKYRPWEKFDFEQVRKSPKPISLLLSTRRRKRNKGWSKDEGTEAEIRKVMNGDYQTSYIEVKRGSKIGEKSAWMLNLSIDVPKIDKGVDPSIIGGIDVGVKSPLVCAINNAFSRYSISDNDLFHFNKKMFARRRILLKKNRRRRAGHGAKNKLKPITILTEKSVRFRKKLIERWACEIADFFIKNKVGTVQIENLESMKRKEDSYFNIRLRGFWPYAEMQNKIEFKLKQYGIEIRKVAPNNTSRTCSKCGHLNNYFNFEYRRKNKFPHFKCEKCNFKEDADYNAALNISNPKLKNTKEEP

SEQ ID NO: 698 - protein, 726 aa, synthetic construct
SEVEFSHEYWMRHALTLAKRARDEREVPVGAVLVLNNRVIGEGWNRAIGLHDPTAHAEIMALRQGGLVMQNYRLIDATLYVTFEPCVMCAGAMIHSRVGRVVFGVRNSKHGAAGSLMNVLNYPGMNHRVEITEGILADECAALLCDFYRMPRRVFNARKKAQSSIDPGGTSGGSSGSETPGTSECATPESSGGRSGGSAKNTITKTLKLRIVRPYNSAEVEKIVADEKNNREKIALEKNKDKVKEACSEHLKVAAYCTTQVERNACLFCKARKLDDKFYQKLRGQFPDAVFWQEISEIFRQLQKQAAEIYNQSLIELYYEIFIKGKGFANASSVEHYLSDVCYTRAAELFKNAAIASGLRGKVKSNFRLKELKNMKSGLPTTKSDNFPIPLVKQKGGQYTGFEISSHNDDFIIKIPFGRWQVKKEIDKYRPWEKFDFEQVRKSPKPISLLLSTQRRKRNKGWSKDEGTEAEIRKVMNGDYQTSYIEVKRGSKIGEKSAWMLSLSIDVPKIDKGVDPSIIGGIDVGVKSPLVCAINNAFCRYSISDNDLFHFNKKMFARRRILLKKSRHRRAGHGAKNKLKPISILTEKSKRFRKKLIERWACEIADFFIKNKVGTVQMENLESMKRREDSYFNIRLRGFWPYAEMQNKIEFKLKQYGIEIRKVAPNNTSKTCSKCGHLNSYFNFEYRKKNKFPHFKCEKCNFKENADYNAALNISNPKLKGTKEEP

SEQ ID NO: 699 - protein, 725 aa, synthetic construct
SEVEFSHEYWMRHALTLAKRARDEREVPVGAVLVLNNRVIGEGWNRAIGLHDPTAHAEIMALRQGGLAMQNYRLVDATLYVTFEPCVLCAGAMVHSRIGRVVFGVRNSKRGAAGSLMNVLNHPGMNHRVEITGGILADECAALLCDFYRMPRQVFNAQKKARSNINSGGSSGGSSGSETLGTSESVTPESSGGSSGGSAKDTITKTLKLRIVRPYNSAEVEKVVADEKNNREKIAMEKNKDKVKEACSKHLKVASYCTTLVERNACPFCKARKLDDKFYQKLRGQFPDAVFWQEIGEIFRQLQKQAAEIYNQSLIELYYEIFIKGKGFANASSVEHYLSDVCYARAAELFKNAAIASGLRGKVKSNFRLKELKNMKSGLPTTKSDNFPIPLVKQKGGQYTGFEISSHNDDFIIKIPFGRWQVKKEIDKYRPWEKFDFEQVRKSPKPISLLLSTQRRKRNKGWSKDEGTEAEIRKVMNGDYQTSYIEVKRGSKTGEKSAWMLNLSIDVPKIDKGVDPSIIGGIDVGVKSPLVCAINNAFSRYSISDNDLFRFNKKMFARRRILLKKNGHKRAGHGAKNKLKPITIMTEKSKRFRKKLIERWACEIADFFIKNKVGTVQMENLESMKRKEDSYFNIRLRGFWPYAEMQDKIEFKLKQYGIEIRKVAPNNTSKTCSKCGHLNNYFNFEYRKKNKFPHFKCEKCSFKENADYNAALNISNPKLKSTEEP

SEQ ID NO: 700 - protein, 726 aa, synthetic construct
SEVEFSHEYWMRHALTLAKRARDEREVPVGAVLVLNNRVIGEGWNRAIGLHDPTAHAEIMALRQGGLVLQNYRLVDATLYVTFEPCVLCAGAMVHSRIGRVVFGARNSKRGAAGSLMNILNYPGMNHRVEITEGILADECAALLCDFYRMPRQVFNARKKARSNINSGGSSGGSSGSETPGTSESATPESSGGSSGGSAKNTITKTLTLRIVRPYNSAEVEKIVADEKNNREKIALEKNKDKVKEACSEHLKVATYCTTQVERNACLFCKARKLDDKFYQKLRGQFPDAVFWQELGEIFRQLQKQAAEIYNQSLVELYYEIFIKGRGFANASSVEHYLSDVCYTRAAELFKNAAIASGLRGKVKSNFRLKELKNMKSGLPTTKSDNFPIPLVKQKGGQYTGFEISSHNDDFIIKIPFGRWQVKKEIDKYRPWEKFDFEQVRKSPKPISLLLSTQRRKRNKGWSKDEGTEAEIRKVMNGGYQTSYIEVKRGSKTGEKSAWMLNLSIDMPKIDKGVDPSIIGGIDVGVKSPLVCAINDAFSRYSISDNDLFHFNKKMFARRRILLKKNRHKRAGHGAKNKLKPLTILTGKSKRFRKKLIERWACEIAGFFIKNKVGTVQMENLESMKRREDSYFNIRLRGFWPYAEMQNKIEFKLKQYGIEIRKVAPNNTSKTCSKCGHLNNYFNFEYRKKNKFPHFKCEKCNFKENADYNAALNISNPKLKSTKEEP

SEQ ID NO: 701 - protein, 726 aa, synthetic construct
SEVEFSHEYWMRHALTLAKRARDEREVPVGAVLVLNNRVIGEGWNRAIGLHDPTAHAEIMALRQGGLVMQNYRLIDATLYVTFEPCVMCAGAMIHSRIGRVVFGVRNSKHGAAGSLMNVLNYPGMNHRVEITEGILADECAALLCDFYRMPRQVFNGRKKAQSSINSGGSSGGSSGSETPGTSESATPESSGGSSSGSTKNTITKTLKLRIVRPYNSTEVEKIVADEKNNREKIALEKNKDKVKEACSRHLKVAAYCTTQVERNACLFCKARKLDDKFYQKLRGQFPDAVFWQEIGEIFRQLQKQAAEIYNQSLIELYYEIFIKGKGFANASSVEHYLSDVCYARAAELFKNAAIASGLRGKVKSNFRLKELKNMKSGLPTTKSDNFPIPLVKQKGGQYTGFEISSHNDDFIIKIPFGRWQVKEEIDKYRPWEKFDFEQVRKSPKPISLLLSTQRRKRNKGWSKDEGTEAEVRKVMNGDYQTSYIEVKRGSKIGEKSTWMLNLSIDVPKIDKGVDPNIIGGIDVGVKSPLVCAINNALSRYSISDNDLFHFNKKMFARRRILLKKNRHKRAGHGTKNKLKPITILTEKSGRFRKKLIERWACEIANFFIKNKVGTVQMENLESMKRKEDSYFNIRLRGFWPYAEMQNKIEFKLKQYGIRIRKVAPNNTSKTCSKCGHLNNYFSFEYRKKNKFPHFKCEKCNFKENADYNAALNISNPKLMSTKEGP

SEQ ID NO: 702 - protein, 726 aa, synthetic construct
SEVEFSHEYWMRHALTLAKRARDKHEVPVGAVLVLNNRVIGEGWNRATGQNDPTAHAEIMALRQGGLVMQNHRLIDATLYVTFEPCVMCAGAMIHSRIGRVVIGVRNSKRGAAGSLMNVLNHPGMNHRVEITEGILADECAALLCDFYRMPRQVFNAQKRAQSSINSGGSSGGSSGSETPGTSESATPESSGGSSAGSTKDTITKTLKLRIVRPYNSAEVEKIVADEKNNREKIALEKNKDKVKEACSKHLKVAAYCTTQVERNACLFCKARRLDDKFYQKLRGQFPDAVFWQELGEIFRQLQKQAAEIYNQSLIELYYEIFIKGKGFANASSVEHYLSDVCYTRAAELFKNAAIASGLRGKVKSNFRLKELKNMKSGLPTTKSDNFPIPLVKQKGGQYAGFEISSHNDDFIIKIPFGRWQVKKEIDKYRPWEKFDFAQVRRSPKPISLLLSTQRRKRNKGWSKDEGTEAEIRKVMNGDYQTSYIEVKRGSKIGEKSAWMLNLSIDVPKIDKGVDPSVVGGIDVGVKSPLVCAINNAFSRYSISDNDLFHFNKKMFARRRILLKKNRHKRAGHGAKNKLKPLTILTGKSKRFRKKLIERWACEIADFFIKNKVGTVQMENLESMKRKEDSYFNIRLRGFWPYAEMQNKIEFKLKQYGIEIRKVAPNNTSKTCSKCGHLNNYFNFEYRKKNKFPHFKCEKCNFKENADYNAALNISNPKLKGTKEEP

SEQ ID NO: 703 - protein, 726 aa, synthetic construct
SEDEFSHEYWMRHALTLAKRARDEREVPVGAILVLNNRVIGEGWNRAIGLHDPTAHAEIMALRQGGLVMQNYRLIDATLYVTFEPCVMCAGAMIHSRIGRVVFGVRNSKHGAAGSLMNVLNYPGMNHRVEITEGILADECAALLCDFYRMPHQVFSARKKAQSSINPGGSSGGSSGSKTPGTSESATPESSGGSSGGSAKNSITKTLKLRIVRPYNSAEVEKIVADEKNNREKIALEKNKDKVKEACSKHLKVASYCTTQVERNACPFCKARKLDDKFYQKLRGQFPDAVFWQELGEILRQLQKQAAEIYNQSLIELYYEIFIKGRGFANASSVEHYLSDVCYTRAAELFKNAAIASGLRGKVKGNFRLKELKNMKSGLPTTKSDNFPIPLVKQKGGQYTGFEISSHNDDFIIKIPFGRWQVKKEIDKYRPWEKFDFEQVRKSPKPISLLLSTQRRKRNKGWSKDEGTEAEIRKVMNGDYQTSYIEVKRGSKTGEKSAWMLNLSIDVPKIDKGVDPSIIGGIDVGVKSPLVCAINNAFSRYSISDNDLFHFNKKMFARRRILLKKSKHKRAGHGAKNKLKPISILTEKSERFRKKLIERWACEIADFFVKNKVGTVQMENLESMKRREDSYFNIRLRGFWPYAKMQNKIEFKLKQYGIEIRKVAPNNTSKTCSKCGHLNNYFNFEYRKKNKFPHFKCEKCNFKENADYNAALNISNPKLKSTKEEP

SEQ ID NO: 704 - protein, 726 aa, synthetic construct
SEVEFSHEYWMRRALTLAKRARDEREVPVGAVLVLNNRVIGVGWNRAVGLHDPTAHAEIMALRQGGLVMQNYRLIEATLYVTFEPCIMCAGAMIHSRIGRVVFGVRNSKRGAAGSLMNVLNYPGMNHRVEITEGILADECAALLCDYYRMPRQVFNARKKAQPSTNSGGPSDGGSGSETPGTSESATPESSGGSSGGSAKNTITKALKLRIVRPYNSAEVEKIVADEKNNRERIALEKNKDKVKEACSKHLKVAAYCTTQVERNACLFCKARKLDDKFYQKLRGQFPDAVFWQEIGEIFRQLQKQAAEIYNQSLIELYYEIFIKGKGFANASSVEHYLSDVCYTRAAELFKNAAIASGLRGKVKSNFRLKELKNMRSGLPTTKSDNFPIPLVKQKGGQYAGFEISSHNDDFIIKIPFGRWQVKKEIDKYRPWEKFDFAQVRKSPKPISLLLSTQRRKRNRGWSKDESTEAEIRKVMNGDYQTSYIEVKRGSKIGEKSAWMLNLSIDVPKIDKGVDPSIVGGIDVGVKSPLVCAINNALSRYSISDNDLFHFNKRMFARRRILLKKNRHKRAGHGAKNKLKPITILTEKSKRFRKKLIERWACEIADFFIKNKVGIVQMENLESMKRREDSYFNIRLRGFWPYAEMQNKIEFKLKQYGIEIRKVAPNNTSKTCSRCGHLNNYFNFEHRKKNKFPRFKCEKCNFKENADYNAALNISNPKLKSTKEEP

SEQ ID NO: 705 - protein, 726 aa, synthetic construct
SEVEFSHEYWMRHALTLAKRARDEREVPVGAILVLNNRVIGEGWNRAIGQHDPTAHAEIMALRQGGLVMQNYRLANATLYVTFEPCVMCAGAMIHSRIGRVVFGVRNSKRGAAGSLMNVLNYPGMNHRVEITEGILTDECAALLCDFYRMPHQVLNAQKKAQSSINSGGSAGGSSGSETPGTSGSTTPVSSGGSSGGSAKNTITKTLKLRIVRPYNSAEVEKIVADEKNNREKTALEKNKDKVKEACSKHLKVASYCTNQVERNACLFCKARKLDDKFYQRLRGQFPDAVFWQELGEIFRQLQKQAAEIYNQSLIELYYEIFIKGKGFANASSVEHYLSDVCYTRAAELFKNAAIASGLRGKVKSNFRLKELKNMKSGLPTTKSDNFPIPLVKQKGGQYTGFEISSHNDDFIIKIPFGRWQVKKEIDKYRPWEKFDFEQVRKSPKPISLLLSTQRRKRNKGWSKDEGTEAEVRKVMNGDYQTSYIEVKRGSKTGEKSAWMLNLSIDVPKIDKGVDPCIIGGIDVGVKSPLVCAINNAFSRYSISDNDLFHFNKKMFARRRILLKENGHKRAGHGAKNKLKPITIMTEKSKRFRKKLIERWACEIADFFIKNKVGIVQMENLESMKRREDSYFNIRLRGFWPYAEMQNKIEFKLKQYGIEIRKVAPNNTSKTCSKCGHLNNYFNFEYRKKNKFPHFKCEKCNFKENADYNAALNISNPRLKSTKEEP

SEQ ID NO: 706 - protein, 726 aa, synthetic construct
SEVEFSHEYWMRHALTLAKRARDEREVPVGAVLVLNNRAIGEGWNRAIGLHDPTAHAEIMALRQGGLVMQNHRLVDATLYVTFEPCVLCAGALVHSRIGRVVFGVRNSKRGAAGSLMNVLNHPGMNHRVEITEGILADECAALLCDFYRMPRQLFNAQKKARSNINSGGSSGGSSGSETPGTSESATPESSGGSSGGSAKNTITKTLKLRIVRPYNNAEVEKIVADEKNNREKTALEKNKDKVKEACSKHLKVAAYCTTQVERNACLFCKARKLDDRFYQKLRGQFPDAVFWQEVGEIFRQLQKQAAEIYNQSLIELYYEIFIKGKGFANASSVEHYLSDVCYTRAAELFKNAAIASGLRGKVKSNFRLKELKNMKSGLPTTKSDNFPIPLVKQKGGQYTGFEISNHNSDFIIKIPFGRWQVKKEINKYRPWEKFDFEQVRKSPKPISLLLSTQRRKRNKGWSKDEGTEAEIRKVMNGDYQTSYIEVKRGSRIGEKSAWMLSLSIDVPKIDRGVDPSIIGGIDVGVKSPLVCAINNSSSRYSISDNDLFHFNKKVFARRRILLKKNRHRRAGHGAKNKLKPITILTEKSKRFRKKLIERWACEIADFFIKNKVGTVQMENLESMKRKEDSYFNIRLRGFWPYAEMQNKIEFKLKQYGIKVRKVAPNNTSRTCSECGHLNNYFSFEYRKKNKFPHFKCKKCNFKEDADYNAALNISNPKLKGTKEEL

SEQ ID NO: 707 - protein, 726 aa, synthetic construct
SEVEFSHEYWMRHALTLAKRARDEREVPVGAVLVLNNRVIGEGWNRAIGLHDPTAHAEIMALRQGGLVMQDYRLIDATLYVTFEPCVMCAGAMVHSRIGRVVFGVRNSKRGAAGSLMNVLDYPGMGHRVEITEGILADECAALLCDFYCMPRQVFNAQKRAQSSINSGGSSGGSSGSETPGTSESATPESSGGSSGGSAKNTITKTLKLRIVRPYNSAEVEKIVADEKNNREKIALEKNKGKVKEACSKHLKVAAYCTTQVERNACLFCKARKLDDKFYQKLRGQFPDAVFWQEIGEIFRQLQKQAAEIYNQSLIELYYEIFIKGKGFANASSVEHYLSDVCYTRAAELFKNAAIASGLRGKVKSNFRLKELKNMKSGLPTTKSDNFPIPLVKQKGGQYTGFEISSHNDDFIIKIPFGRWQVKKEIDKYRPWEKFDFEQVRKSPKPISLLLSTQRRKRNKGWSKDEGTEAEIRKVMNGDYQTSYIEVKRGSKTGEKSAWMLNLSIDVPKIDKGVDPSIIGGIDVGVKSPLVCAINNAFSRYSISDNDLFHFNKKVFARRRILLKKNKHKRAGHGAKNKLKPITILTEKSGRFRKKLIERWACEIADFFIKNKVGTVQMENLESMKRKEDSYFNIRLRGFWPYAEMQNKIEFKLKQYGIVVRKVAPNNTSKTCSKCGHLNNYFNFEYRKKNKFPHFKCEKCNFKENADYNAALNISNPKLKSTKEEP

SEQ ID NO: 708 - protein, 726 aa, synthetic construct
SEIEFSHEYWMRHALTLARRARDEREVPVGAILVLNNRVIGEGWNRAIGLHDPTAHAEIMALRQGGLVMQNYRLTDATLYVTFEPCVMCAGAMIHSRIGRVVFGVRNSKHGAAGSLVNVLNYPGMNHRVEITEGVLADECAALLCDFYRMPRQVFNARKKAQSSINPGGSSGGSSGSETPGTSESATLENSGGSSGGSAKNTITKTLKLRIVRPYNSAEVEKIVADEKNNREKIALEKNKDKVKEACSKHLKVAAYCTTQVERNACLFCKARRLDDKFYQKLRGQFPDAVFWQEIGEILRQLQKQAAEIYNQSLIELYYEIFIKGRGFANASSVEHYLSDVCYTRAAELFKNAAIASGLRGKVKSNFRLKELKNMKSGLPTTKSDNFPIPLVKQKGGQYTGFEISSHNDDFIIKIPFGRWQVKKEIDKYRPWEKFDFEQVRKSPKPISLLLSTQRRKRNKGWSKDEGTEAEIRKVMNGDYQTSYIEVKRGSKVGEKSAWMLSLSIDVPKIDKGVNPSIIGGIDVGVKSPLVCAINNALSRYSVSDNDLFRFNKKMFARRRILLKKNRHKRAGHGAKNKLKPITILTKKSERFRKKLIERWACEIADFFIKNKVGTVQMENLESMKRKEDSYFNIRLRGFWPYAEMQNKIEFKLKQYGIEIRKVAPNNTSKTCSKCGHLNNYFNFEYRKRNKFPHFKCEKCNYKEDADYNAALNISNPKLKSTKEEP

SEQ ID NO: 709 - protein, 726 aa, synthetic construct
SEVEFSHEYWMRHALTLAKRARDEREVPVGAILVLNNRVIGEGWNRAIGLHDPTAHAEIMALRQGGLVMQNYRLTDATLYVTFEPCVMCAGAMIHSRIGRVVFGVRNSKHGAAGSLMNVLNYPGMNHRVEITEGILVDECAALLCDFYRMPRQVFNARKKAQSNIHPGGSSGSSSGSETPGTSKSATPGSSGGSTGGSAKNTITKTLTLRIVRPYNSAEVEKIVADEKNNREKIALEKNKDKVKEACSEHLKVAAYCTTQVEKSACLFCKARKLDDKFYQKLRGQFPDAVFWQEIGEIFRQLQKQAAEIYNQSLIELYYEIFIKGKGFANASSVEHYLSDVCYTRAAELFKNAAIASGLRGKVKSNFRLKELKNMKSGLPTTKSDNFPIPLVKQKGGQYTGFEISSHNDDFIIKIPFGRWQVKKEIDKYRPWEKFDFEQVRKSPKPISLLLSTRRRKRNKGWSKDEGTEAEIRRVMNGNYQTSYIEVKRGSKIGEKSAWMLNLSIDVPKIDKGVDPSIIGGIDVGVKSPLVCAINNAFSRYSIGDNELFHFNKKMFARRRILLKKNRHKRAGHGVKNKLKPITTLTEKSRRFRKKLIERWACEIADFFVKNKVGTVQMENLESMKRKEDSYFNIRLRGFWPYAEMQNKIEFKLEQYGIVVRKVAPNNTSKTCSKCGHLNNYFNFEYRKKNKFPHFKCEKCSFKENADYNAALNISNPKLKGTKEEP

SEQ ID NO: 710 - protein, 726 aa, synthetic construct
SEVEFSHEYWMRHALTLAKRARDEREVPVGAILVLNNRVIGEGWNRAIGLHDPTAHAEIMALRQGGLVMQNYRLIDATLYVTFEPCVMCAGAMVHSRIGRVVFGVRNSKRGAAGSLMNVLDYPGMDHRVEITEGILADECAALLCDFYRMPHQVFNAQKKAQSSINPGGSSGGSSGSETPGTSESATPESSGGSSGGSAKNTITKALKLRIVRPYNSAEVEKIVADEKNNREKIALEKNKDKVKEACSKHLKVATYCTTQVERNACLFCKARKLDDKFYQKLRGQFPDAVFWQEIGEIFRQLQKQAAEIYNQSLVELYYEIFIKGKGIANASSVEHYLSDVCYTRAAELFKNAAIASGLRNKIKSNFRLKELRNMKSGLPTTKSDNFPIPLVRQKGGQYTGFEISNHNGDFIIKIPFGRWQVKKEICKHRPWEKFDFEQVRKSPKPISLLLSTQRRKRNKGWGKDEGTEAEIRKVMNGDYQTSYIEVKRGSKIGEKSAWMLNLSIDVPKIDKGVDPSIIGGIDVGVKSPLVCAINNALSRYSISDNDLFHFNKKMFARRRILLRKNRHKRAGHGARNKLKPITVLTEKSERFRKKLIERWACEIANFFIKNKVGTVQMENLESMKRREDSYFNVRLRGFWPYAEMQNKIEFKLKQYGIVVRKVAPNNTSKTCSRCGHLNDYFNFEYRKKNKFPRFKCEKCNLKEDADYNAALNISNPKLKSTKEEP

SEQ ID NO: 711 - protein, 726 aa, synthetic construct
SEVEFSHEYWMRHALTLARRARDEREVPVGAVLVLNNRVIGEGWNRAIGLHDPTAHAEIMALRQGGLVMRNYRLTDATLYVTFEPCVMCAGAMIHSRIGRVVFGVRNSKRGAAGSLMNVLNYPGMNHCVEITEGILVDECAALLCDFYRMPRQVLNAQKKAQSSISPGGSSGGSSGSETPGASESVTPKSSGGSSGGSAKNTITKTLKLRIVRPYNSAEVEKIVADEKNNREKIALEKNKGKVKEACSKHLEVAAYCTTQVERNACLFCKARKLDDKFYQKLRGQFPDAVFWQELGEIFRQLQKQAAEIYNQSLIELYYEIFIKGRGFANAGSVEHYLSDVCYTRAAEQFKNAAIASGLRGKVKSNFRLKELKNMKSGLPTTKSDNFPIPLVKQKGGQYTGFEISSHNDDFIIKIPFGRWQVKKEIDKYRPWEKFDFEQVRKSPKPISLLLSTQRRKRNKGWSKDEGTEAEIRKVMNGDYQTSYIEVKRGSKTGEKSAWMLNLSIDVPKIDKGVDPCIIGGIDVGVKSPLVCAINNAFSRYSISDNDLFHFNKKMFARRRILLKENGHKRAGHGAKNKLKPITIMTEKSKRFRKKLIERWACEIADFFIKNKVGTVQMENLESMKRKEDSYFNIRLRGFWPYAEMQNKIEFKLKQYGIVVRKVAPNNTSKTCSECGHLNNYFNFEYRKKNKFPLFKCEKCNFKENADYNAALNISNPKLKSTKGEP

SEQ ID NO: 712 - protein, 726 aa, synthetic construct
SEVEFSHEYWMRHALTLAKRARDEREVPVGAVLVLNNRVIGEGWNRAIGLHDPTAHAEIMALRQGGLVMQNYRLTDATLYVTFEPCVMCAGAMIHSRIGRVVFGVRNSKRGAAGSLMNVLNYPGMNHCVEITEGILVDECAALLCDFYRMPRQVLNAQKKAQSSISPGGSSGGSSGSETPGASGSVTPKSSGGSSAGSTKVTITKTLKLRIVRPYNSAEVEKIVADEKNSREKIALEKNKDKVKEACSEHLKVAAYCTTQVERNACLFCKARKLDDRFYQKLRGQFPDAVFWQEIGEIFRQLQKQAAEIYNQSLIELYYEIFIKGKGFANASSVEHYLSDVCYTRAAELFKNAAIASGLRGKVKSNFRLKELKNMKSGLPTTKSDNFPIPLVKQKGGQYTGFEISNHNSDFIIKIPFGRWQAKKEIDRYRPWERFDFEQVRRSPKPISLLLSTQRRKRNKGWSKDEGTEAEIRKVMNGDYQTSYIEVKRGSKIGEKSAWMLNLSVDVPKIDKGIDPSIIGGIDVGVKSPLVCAINNAFGRYSISDNDLFHFNKKMFARRRILLKKNRHKRAGHGAKNKLKPITILTEKSKRFRKKLIERWACEIADFFVKNKVGTVQMENLESMKRKEDSYFNIRLRGFWPYAEMQNKIEFKLKQYGIKVRKVAPNNTSKTCSKCGHLNNYFSFEYRKKNKFPHFKCEKCNFKENADYNAALNISNPKLKSTKEEP

SEQ ID NO: 713 - protein, 726 aa, synthetic construct
SEVEFSHEYWMRHALTLAKRARDEREVPVGAVLVLNNRVIGEGWNRAIGLHDPTAHAEIMALRQGGLVMQNYRLTDATLYVTFEPCVMCAGAMIHSRIGRVVFGVRNSKRGAAGSLMNVLSYPGMNHCVEITEGILVDECAALLCDFYRMPRQVLNAQKKAQSSISSGGSSGGSSGSETPGASESVTPRSSVGSSASSTKNTITKTLKLRIVRPYNSAEVEKIVADEKNNREKIALEKNKDKVREACSKHLKVASYCTTQVERNACPFCKARKLDDKFYQKLRGQFPDAVFWQELGEIFRQLQKQAAEIYNQSLIELYYEIFIKGKGFANASSVEHYLSDVCYTRAAELFKNAAIASGLRGKVKSNFRLKELKNMKSGLPTTKSDNFPIPLVKQKGGQYTGFEISSHNDDFIIKIPFGRWQVKKEIDKYRPWEKFDFEQVRKSPKPISLLLSTQRRKRNKGWSKDEGTEAEIRKVMNGDYQTSYIEVKRGSKIGEKSAWMLNLSIDVPKIDKGVDPSIIGGIDVGVKSPLVCAINNAFSRYSISDNDLFRFNKKMFARRRILLKKNRHKRAGHGAKNKLKPITILTGKSRRFRKKLIERWACEIADFFIKNKVGTVQMESLESMKRKEDSYFNIRLRGFWPYAEMQNKIEFKLKQYGIEIRKVAPNNTSKTCSKCGHLNNYFNFEFRKKNKFPHFKCEKCNFKENADYNAALNISNPKLKSTKEEP

SEQ ID NO: 714 - protein, 726 aa, synthetic construct
SEVEFSHEYWMRHALTLAKRARDEREVPVGAILVLNNRVIGEGWNRAIGLHDPTAHAEIMALRQGGLVMQNYRLTDATLYVTFEPCVMCAGAMIHSRIGRVVFGVRNSKRGAAGSLMNVLNYPGMNHCVEITEGILVDECAALLCDFYRMPRQVLNAQKKAQSSISSGGSSGGSSGSETPGASGSVIPKSSGGSSAGSTKDTITKTLKLRIVRPYNSAEVEKIVADEKNNREKIALEKNKDKVKEACSKHLKVAAYCTTQVERNACLFCKARKLDDKFYQKLRGQFPDAVFWQEIGEIFRQLQKQAAEIYNQSLIELYYEIFIKGKGFANASSVEHYLSDVCYTRAAELFKNAAIASGLRGKVKSNFRLKELKNMKSGLPTTKSDNFPIPLVKQKGGQYTGFEISSHNDDFIIKIPFGRWQAKKEIDKYRPWEKFDFEQVRKNPKPISLLLSTQRRKRNKGWSKDEGTEAEIRKVMNGDYQTSYIEVKRGSKIGEKSAWMLNLSIDVPKIDKGVDPGIIGGIDVGVKSPLVCAINNAFSRYSISDNDLFRFNKKVFARRRILLEKNRHKRAGHGVKNKLKPITILTEKSRRFRKKLIERWACEIADFFVKNKVGTVQMENLEGMKRKEDSYFNIRLRGFWPYAEMQNKIEFKLKQYGIKVRKVAPNNTSKTCSKCGHLNNYFSFEYRKKNKFPHFKCEKCNFKENADYNAALNISNPKLKSTKEEP

SEQ ID NO: 715 - protein, 726 aa, synthetic construct
SEVEFSHEYWMRHALTLAKRARDEREVPVGAVLVLNNRVIGEGWNRAIGLHDPTAHAEIMALRQGGLVLQNYRLVDATLYVTFEPCVLCAGAMVHSRIGRVVFGARNSKRGAAGSLMNILNYPGMNHRVEITEGILADECAALLCDFYRMPRQVFNAQKKAQSSINSGGSPGGSSGSETPSTSESATPESSGGSSGGSAKNTITKTLQLRIVRPYNSAEVEKIVTDEKNNREKIALEKNKDKVKEACSKHLKMASYCTTQVERNACLFCKARKLDDKFYQKLRGQFPDAVFWQELGGIFRQLQKQAAEIYNQSLIELYYEIFIKGKGITNASRVEHYLSDVCYTRAAELFKNAAIASGLRSKVRSNFRLKELKNMKSGLPTTKSDNFPIPLVKQKGGQYTGFEVSSHNSDFIIKIPFGRWQVKEEIDKYRPWEKFDFEQVRKSPKPISLLLSTQRRKKNKGWSKDEGTEAEIRRVMNGDYRTSYIEVKRGSKIGEKSAWMLNLSIDVPKIDKGVDPSIIGGIDVGVKSPLVCAINNSSSRYSICDNDLFRFNKKMFARRRILLKKNRHKRAGHGAKNKLKPITILTKKSERFRKKLIERWACEIADFFIKNKVGTVQMENLESMKRKEDSYFNIRLRGFWPYAEMQNKIEFKLKQYGIEIRKVAPNNTSKTCSKCGHLNNYFNFEYRRKNKFPHFKCEKCNFKENADYNAALNISNPKLKSTKEEP

SEQ ID NO: 716 - protein, 726 aa, synthetic construct
SEVEFSHEYWMRHALALAKRARDEREVPVGAVLVLNNRAIGEGWNRAIGLHDPTAHAEIMALRQGGLVMQNYRLTDATLYVTFEPCVMCAGAMIHSRIGRVVFGVRNSKRGAAGSLMNVLNYPGMNHCVEITEGILVDECAALLCDFYRMPRQVLNAQKKAQSSISSGGSSGGSSGSETPSTSESATPESSGGSSGGSAKNTITKTLQLRIVRPYNSAEVEKIVTDEKNNREEIALEKNKDKVKEACSKHLKMASYCTTQVERNACLFCKARKLDDKFYQKLRGQFPDAVFWQELGGIFRQLQKQAAEIYNQSLIELYYEIFIKGRGFANASSVEHYLSDVCYTRAAELFKNAAIASGLRGKVKSNFRLKELKNMKSGLPTTKSDNFPIPLVKQKGGQYTGFEISSHNDDFIIKIPFGKWQVKKEIDKYRPWEKFDFEQVRKSPKPISLLLSTQRRKRNKGWSKDEGTEAEIRKVMNGDYQTSYIEVKRGSKTGEKSAWMLNLSIDVPKIDKGVDPSIIGGIDVGVKSPLVCAINNAFSRYSISDNELFHFNKKMFARRRILLKKNRHKRAGHGVKNKLKPISILTEKSERFRKKLIEKWACEIADFFIKNKVGTVQMENLESMKRKEDSYFNIRLRGFWPYAEMQNKIEFKLKQYGIEIRKVAPNNTSKTCSKCGHLNNYFNFEYRKKNKFPHFKCEKCNFKENADYNAALNISNPKLKSTKEGP

SEQ ID NO: 717 - protein, 726 aa, synthetic construct
SEVEFSHEYWMRHALTLAKRARDEREVPVGAILVLNNRVIGEGWNRTAGLHDPTAHAEIMALRQGGLVMQNHRLVDATLYVTFEPCVMCAGAMIHSRIGRVVFGVRNSKRGAAGSLTNVLNYPGMNHCVEVTEGILVDECAALLCDFYRMPRQVLNAQKKAQSSISPGGSSGGSSGSETPGASESVTPKSSGGSSGGSAKNTITKTLKLRIVRPYNSAEVEKIVADEKNNREKIALEKNKDKVKEACSKHLKVASYCTTQVERNACLFCKARKLDDKFYQKLRGQFPDAVFWQELGEIFRQLQKQAAEIYNQSLVELYYEIFVKGKGFANASSVEHYLSDVCYTRAAELFKNAAIASGLRGKVKSNFRLKELKNMKSGLPTTKSDNFPIPLVKQKGGQYTGFEISSHNDDFIIKIPFGRWQVKKEIDKYRPWEKFDFEQVRKSPKPISLLLSTQRRKRNKGWSKDEGTEAEIRKVMNGDYQTSYIEVKRGSKIGEKSAWMLNLSIDVPKIDKGVDPSIVGGIDVGVKSPLVCAINNAFSRYSISDNDLFHFNKKMFARRRILLKKSKHKRAGHGAKNKLKPITILTEKSGRFRKKLIERWACEIADFFIKNKVGTVQMENLEGMKRKEDSYFNIRLRGFWPYAEMQNKIEFKLKQYGIEIRKVAPNNTSKTCSKCGHLNNYFNFEYRKKNKFPHFKCEKCNFKENADYNAALNISNPKLKSTKEEP

SEQ ID NO: 718 - protein, 726 aa, synthetic construct
SEVEFSHEYWMRHALTLAKRARDEREVPVGAVLVLNNRVIGEGWNRTTGLHDPTAHAEIMALRQGGLVMRNYRLTDATLYVTFEPCVMCAGAMIHSRIGRVVFGVRNSKRGAAGSLMNVLNYPGMNHRVEITEGILADECAALLCDFYRMPRQVFNAQKKARSNINSGGSSGGSSGSETPGTSESTTRESSGGSSGGSAKNTITKTLKLRIVRPYNSAEVEKIVADEKNNREKIAMEKNKDKVKEACSKHLKVASYCTTQVERNACLFCKARKLDDKFYQKLRGQFPDAVFWQEVGEIFRQLQKQAAEIYNQSLVELYYEIFIKGKGIANASSVEHYLSDVCYTRAAELFKNAAIASGLRGKVKSNFRLKELKNMKSGLPTTKSDNFPIPLVKQKGGQYTGFEISSHNDDFIIKIPFGRWQAKKEIDKYRPWEKFDFEQVRKSPKPISLLLSTQRRRRNKGWSKDGGTEAEIRKVMNGDYQISYIEVKRGNKIGEKSAWMLNLSIDVPKIDKGVDPSIIGGIDVGVKSPLVCAINNALSRYSISDNDLFRFNKKMFARRRILLKKNGHKRAGHGAKNKLKPITIMTEKSKRFRKKLIERWACEIADFFIKNKVGTVQMENLESMKRKEDSYFNIRLRGFWPYAEMQNKIEFKLKQYGIVVRKVAPNNTSKTCSQCGHLNNYFNFEHRKKNKFPHFKCEKCNFKENADYNAALNISNPKLKSTKGEP

SEQ ID NO: 719 - protein, 726 aa, synthetic construct; identical to SEQ ID NO: 563

SEQ ID NO: 720 - protein, 726 aa, synthetic construct
SEVEFSHEYWMRHALTLAKRARDEREVPVGAVLVLNNRVIGEGWNRAIGLHDPTAHAEIMALRQGGLVMQNYRLIDATLYVTFEPCVMCAGAMIHSRIGRVVFGVRNNKRGAAGSLMNVLNYPGMNHRVEITEGILADECAALLCDFYRMPRQVLNAQKKARSCINPGGSSGGSSGSETPGTSESATPESSGGGSSGSAKNTITKTLQLRIVRPYNSAEVEKIVADEKNNRERIALEKNKDKVREACSKHLKVASYCTTQVERNACPFCKARKLDDKFYQKLRDQFPDAVFWQEIGEIFRQLQKQAAEIYNQSLIELYYEIFIKGKGFANASSVEHYLSDVCYTRAAELFKNAAIASGLRGKVKSNFRLKELKNMKSGLPTTKSDNFPIPLVKQKGGQYTGFEISSHNDDFIIKIPFGRWQVKKEIDKYRPWEKFDFEQVRKSPKPISLLLSTQRRKRNKGWSKDEGTEAEIRKVMNGDYQTSYIEVKRGSKIGEKSAWMLNLSIDVPKIDKGVDPSIIGGIDVGVKSPLVCAINNAFSRYSIGDNDLFHYNKKMFARRRILLKKNRHKRAGHGAKNKLKPISILTEKSKRFRKKLIERWACEIADFFIKNKVGTVQIENLESMKRKEDSYFNIRLRGFWPYAEMQNKIEFKLKQYGIKVRKVAPNNTSKTCSKCGHLNNYFSFEYRKKNKFPHFKCEKCDFKENADYNAALNISNPKLKSTKEEP

SEQ ID NO: 721 - protein, 726 aa, synthetic construct
SEVEFSHEYWMRHALTLAKRARDEREVPVGAVLVLNNRVIGEGWNRAIGLHDPTAHAEIMALRQGGLVMQNYRLTDATLYVTFEPCVMCAGAMIHGRIGRVVFGVRNSKRGAAGSLMNVLSYPGMNHCVEITEGILVDECAALLCDFYRMPRQVFNARKKAQSSINPGGSSGGSSGSETPGTSESATPESSGGSSGGSAKNTITKALKLRIVRPYNSAEVEKIVADEKNIREKIALEKNKDKVKEACSKHLKVASYCTTQVERNACPFCKARKLDDKFYQKLRGQFPDAVFWQEIGEIFRQLQKQAAEIYNQSLIELYYEIFIKGKGFANASSVEHYLSDVCYTRAAELFKNAAIASGLRGKVKSNFRLKELKNMKSGLPTTKSDNFPIPLVKQKGGQYTGFEISSHNDDFIIKIPFGRWQVKKEIDKYRPWEKFDFEQVRKSPKPISLLLSTQRRKRNKGWSKDEGTEAEIRKVMNGDYQTSYIEVKRGSKTGEKSAWMLNLSIDVPKIDKGVDPSIIGGIDVGVKSPLVCAINNAFSRYSISDNDLFRFNKKMFARRRILLKKNRHKRAGHGAKNKLKPISILTGKSERFRKKLIERWACEIADFFIKNKVGTVQMENLESMKRKEDSYFNIRLRGFWPYAEMQNKIEFKLKQYGIEIRKVAPNNTSKTCSKCGHLNNYFNFEYRKKNKFPHFKCEKCNFKENADYNAALNISNPKLKSTKEEP

SEQ ID NO: 722 - protein, 726 aa, synthetic construct
SEVEFSHEYWMRHALTLAKRARDEREVPVGAILVLNNRVIGEGWNRAIGLHDPTAHAEIMALRQGGLVMQNYRLIDATLYVTFEPCVMCAGAMIHSRIGRVVFGVRNNKHGAAGSLVNVLNYPGMNHRVEITEGILADECAALLCDFYRMPRQVFNARKKAQSSTNPGGSSGGSSGSETPGTSESPTPGSSGGSSGGSAKNTITKTLKLRIVRPYNSAEVEKIVAEEKNNREKIALEKNKDKVKEACSKHLKVASYCTTQVERNACLFCKARKLDDKFYQKLRGQFPDAVFWQELGEIFRQLQKQAAEIYNQSLIELYYEIFIKGKGFANASSVEHYLSDVCYTRAAELFKNAAIASGLRGKVKSNFRLKELKNMKSGLPTTKSDNFPIPLVKQKGGQYTGFEISSHNDDFIIKIPFGRWQVKKEIDKYRPWEKFDFEQVRKSPKPISLLLSTQRRKRNKGWSKDEGTEAEIRKVMNGDYQTSYIEVKRGSKIGEKSAWMLNLSIDVPKIDKGVDPNIIGGIDVGVKSPLVCAINNAFNRYSISDNNLFHFNKKMFARRRILLKKNRHKRAGHGAKNKLKPISILTEKSERFRKKLIERWACEIADFFIRNKVGTVQMENLESMKRKEDSYFNIRLRGFWPYAEMQNKIEFKLKQYGIEVRKVAPNNTSKTCSKCGHLNNYFNFEYRKKNKFPHFKCEKCNFKENADYNAALNISNPKLKSTKEEH

SEQ ID NO: 723 - protein, 726 aa, synthetic construct
SEVEFSHEYWMRHALTLAKRARDEREVPVGAILVLNNRVIGEGWNRAIGLNDPTAHAEIMALRQGGLVMQNYRLIDATLYVTFEPCVMCAGAMIHSRIGRVVFGVRNNKHGAAGSLVNVLNYPGMNHRVEITEGILADECAALLCDFYRMPRQVFNARKKAQSSINPGGSSGGSGGSETPGTSECPTPESSGGSSGGSAKNTITKTLKLRIVRPYNSAEVEKIVAEEKDNREKIALEKNKDKVREACSKHLKVAAYCTTQVERNACLFCKARKLDDKFYQKLRGQFPDAVFWQEIGEIFRQLQKQAAEIYNQSLIELYYEIFIKGKGFANASSVEHYLSDVCYTRAAELFKNAAIASGLRGKVKSNFRLKELKNMKSGLPTTKSDNFPIPLVKQKGGQYTGFEISSHNDDFIIKIPFGRWQVKKEIDKYRPWEKFDFEQVRKSPKPISLLLSTQRRKRNKGWSKDEGTEAEIKRVMNGDYQISYIEVKRGSKIGEKSAWMLSLSVDVPKIDKGVDPSIIGGIDVGVKSPLVCAINNALSRYSISDNDLFHFNKKMFARRRILLRNNRHKRAGHGAKSKLKPITILTEKGERFRKKLIERWACEIANFFIKNKVGTVQMENLESMKRKEDSYFNVRLRGFWPYAEMQNKIEFKLKQYGIEIRKVAPNNTSKTCSRCGHLNNYFNFEYRRKNKFPHFKCEKCNFKENADYNAALNISNPKLKSTKEEP

SEQ ID NO: 724 - protein, 726 aa, synthetic construct
SEVEFSHEYWMRHALTLAKRARDEREVPVGAVLVLNNRVIGEGWNRAIGLHDPTAHAEIMALRQGGLVMQNYRLTDATLYVTFEPCVMCAGAMIHSRIGRVVFGVRNSKRGAAGSLMNVLNYPGMNHCVEITEGILVDECAALLCDFYRMPRQVLNAQKKAQSNISSGGPSGGSSCSETPGTSESATPESSGGSSGGSAKNTITKALKLRIVRPYNSAEVEKIVADEKNNREKIALEKNKDKVKEACSKHLKVAAYCTTQVERNACLFCKARRLDDKFYQKLRGQFPDAVFWQEIGEIFRQLQKQAAEVYNQSLVELYYEILIKGKGIANASSVEHYLSDVCYTRAAELFKNAAIASGLRNKIKSNFRLKELRNMKSGLPTTKSDNFPIPLVKQKGGQYTGFEISNHNSDFIIKIPFGRWQVKKEINKYRPWEKFDFEQVRKSPKPISLLLSTQRRKRNKGWSKDEGTEAEIRKVMNGDYQTSYIEVKRGSRIGEKSAWMLSLSIDVPKIDRGVDPSIIGGIDVGVKSPLVCAINNALSRYSISDNDLFHFNKKMFARRRILLKKNRHKRAGHGAKNKLKPLTILTGKSKRFRKKLIERWACEIADFFIKNKVGTVQMENLESMKRKEDSYFNIRLRGFWPYAEMQNKIEFKLKQYGIEIRKVAPNNTSKTCSKCGHLNNYFNFEYRKKNKFPHFKCEKCNFKENADYNAALNISNPMLKSTKEET

SEQ ID NO: 725 - protein, 726 aa, synthetic construct
SEVEFSHEYWMRHALILAKRARDEREVPVGAVLVLNNRVIGVGWNRAVGLHDPTAHAEIMALRQGGLVMQNYRLIEATLYVTFEPCIMCAGAMIHSRIGRVVFGVRNSKRGAAGSLMNVLNYPGMSHRVEITEGILADECAALLCDYYRMPRQVFNARKKAQSSINSGGSSGGSSGSETPGTSESATPKSSGGSSGGSAKNTITKALKLRIVRPYNSAEVEKIVADEKNNRERIALEKNKDKVKEACSKHLKVAAYCTTQVERNACLFCKARKLDDKFYQKLRGQFPDAVFWQEIGEIFRQLQKQAAEIYNQSLIELYYEIFIKGKGFANASSVEHYLSDVCYTRAAELFKNAAIASGLRGKVKSNFRLKELKNMRSGLPTTKSDNFPIPLVKQKGGQYTGFEISSHNDDFIIKIPFGRWQVKKEIDKYRPWEKFDFEQVRKSPKPISLLLSTRRRKRNKGWSKDEGTEAEIRKVMNGDYQTSYIEVKRGSKIGEKSAWMLNLSIDVPKIDKGVDPSIIGGIDVGVKSPLVCAINNAFSRYSISDNELFHFNKKMFARRRILLKKNRHKRAGHGAKNKLKPISVLTEKSGRFRKKLIERWACEIADFFIKNKVGTVQMENLGSMKRKEDSYFNIRLRGFWPYAEMQNKIEFKLKQYGIEIRKVAPDNTSKTCSKCGHLNNYFNFEYRKKNKFPHFKCEKCNFKEDADYNAALNISNPKLKSTKEEP

SEQ ID NO: 726 - protein, 726 aa, synthetic construct
SEVEFSHEYWMRHALTLAKRARDEREVPVGAVLVLNNRVIGEGWNRAIGLHDPTAHAEIMALRQGGLVMQNYRLTDATLYVTFEPCVMCAGAMIHSRIGRVVFGVRNSKRGAAGSLMNVLNYPGMNHCVEITEGILVDECAALLCDFYRMPRQVLSAQKKAQSSISSGGSSGGSSGSETPGASESVTPKSSGGNSGGSAKNTITKTLKLRIVRPYNSAEVEKIVADEKNNREKIALEKNKGKVKEACSKHLEVAAYCTTQVERNACLFCKARKLDDKFYQKLRGQFPDAVFWQELGEIFRQLQKQAAEIYNQSLIELYYEIFIKGKGFANASSVEHYLSDVCYTRAAELFKNAAIASGLRGKVKSNFRLKELKNMKSGLPTTKSDNFPIPLVKQKGGQYTGFEINSHNDDFIIKIPFGRWQVRKEIDKYRPWEKFNFEQVRKSPKPISLLLSTQRRKRNKGWSKDEGTEAEIRKVMNGDYQTSYIEVKRGSKIGEKSAWMLSLSIDVPKIDKGVDPSIIGGIDVGVKSPLVCAINNAFNRYSISDNNLFHFNKKMFARRRILLKKNRHKRAGHGAKNKLKPISILTEKSERFRKKLIERWACEIADFFIRNKVGTVQMENLEGMRGKEDSYFNIRLRGFWPYAEMQNKIEFKLKQYGIEVRKVAPNNTSKTCSKCGHLNNYFNFEYRKKNKFPHFKCEKCNFKENADYNAALNISNPKLKSTKEEP

SEQ ID NO: 727 - protein, 726 aa, synthetic construct
SEVEFSHEYWMRRALTLAKRARDEREVPVGAVLVLNNRVIGVGWNRAAGLHDPTAHAEIMALRQGGLVMQNYRLVEATLYVTFEPCIMCAGAMIHSRIGRVVFGVRNSKRGAAGSLMNVLNYPGMNHRVEITEGILADECAALLCDYYRMPRQVFNARKKAQSSINSGGSSDGGSGSETPGTSESATPESSGGSSGGSAKNTITKTLKLRIVRPYNSAEVEKIVADEKNDREKIALEKNKDKVREACSEHLKVAAYCTTQVERSACLFCKARKLDDKFYQKLRGQFPDAVFWQEIGEIFRQLQRQAAEIYNQSLIELYYEIFIKGKGFANASSVEHYLSDVCYTRAAELFKNAAIASGLRGKVKSNFRLKELKNMKSGLPTTKSDNFPIPLVKQKGGQYTGFEISSHNDDFIIKIPFGRWQVKKEIDKYRPWEKFDFEQVRKSPKPISLLLSTQRRRRNKGWSKDEGTEAEIRKVMNGDYQTSYIEVKRGSKIGEKSAWMLSLSIDVPKIDKGVDPSIIGGIDVGVKSPLVCAINDAFSRYSISDNDLFHFNKKMFARRRILLKKNRHKRAGHGAKNKRKPISILTEKSKRFRKKLIERWACEIADFFIKNKVGTVQMENLESMKRKEDSYFNIRLRGFWPYAEMQSKIEFKLKQYGIEIRKVAPNNTSKTCSKCGHLNNYFNFEYRKKNKFPHFKCEKCNFKENADYNAALNISNPRLKSTKEEP

SEQ ID NO: 728 - protein, 726 aa, synthetic construct
SEVEFSHEYWMRHALTLAKRARDEREVPVGAVLVLDNRVIGVGWNRAIGLHDPTAHAEIMALRQGGLVMQNYRLTDATLYVTFEPCVMCAGAMVHSRIGRVVFGVRNSKRGAAGSLMNVLNYPGMSHCVEITEGILVDECAALLCDFYRMPRQVLNAQKKAQSSISSGGSSGGSGGGETPGASESVTPKNSGGSSAGSTKNTITKTLKLRIVRPYNSAEVEKIVADEKNSREKIALEKNKDKVKEACREHLKVAAYCTTQVERSACLFCKARKLDDRFYQKLRGQFPDAVFWQEISEIFRQLQKQAAEVYNQSLVELYYEILIKGKGIANASSVEHYLSDVCYTRAAELFKNAAIASGLRNKIKSNFRLKELRNMKSGLPTTKSDNFPIPLVKQKGGQYTGFEISSHNDDFIIKIPFGRWQAKKEIDKYRPWEKFDFEQVRKSPKPISLLLSTQRRKRNKGWSKDEGTEAEIRKVMNGDYQTSYIEVKRGSKIGEKSAWMLNLSIDVPKIDKGVDPSIIGGIDVGVKSPLVCAINNAFIRYSISDNDLFHFNKKMFARRRILLKKNRHKRAGHGAKNKLKPISILTEKSKRFRKKLIERWACEIADFFIKNKVGTVQMENLESMKRKEDSYFNIRLRGFWPYAEMQNKIEFKLKQYGIEIRKVAPNNTSRTCSKCGHLNNYFNFEYRKKNKFPHFRCEKCNFKEDADYNAALNISNPKLKSTKEEP

SEQ ID NO: 729 - protein, 726 aa, synthetic construct
SEVEFSHEYWMRHALTLAKRARDEREVPVGAVLVLNNRVIGEGWNRAIGLHDPTAHAEIMALRQGGLVMQNYRLTDAILYVTFEPCVMCAGAMVHSRIGRVVFGVRNSKRGAAGSLMNVLNYPGMNHCVEITEGILVDECAALLCDFYRMPRQVLNAQKKAQSSISPGGSSGGSSGSETPGASESVTPKSSGGSSGGSAKNTITKTLKLRIVRPYNSAEVEKIVADEKNNREKIALEKNKGKVKEACSRHLEVAAYCTTQVERNACLFCKARKLDDKFYQKLRGQFPDAVFWQELGEIFRQLQKQAAEIYNQSLIELYYEIFIKGKGFANASSVEHYLSDVCYTRAAELFKNAAIASGLRGKVKSNFRLKELRNMKSGLPTTKSDNFPIPLVKQKGGQYTGFEISSHNDDFIIKIPFGRWQVRKEIDKYRPWEKFDFEQVRKSPKPISLLLSTQRRRRNKGWSKDEGTEAEIRKVMSGDYQTSYIEVKRGSKIGEKSAWMLSLSIDVPKIDKGVDPRIIGGIDVGVKSPLVCAINNVLSRYSISDNDLFHFNKKMFARRRILLKKNRHKRAGHGAKNKLKPISILTEKSKRFRKKLIERWACEIADFFIKNKVGTVQVENLESMKRKEDSYFNIRLRGFWPYAEMQNKIEFKLKQYGIEIRKVAPNNTSKTCSKCGHLNSYFDFEYRKRNKFPHFKCEKCNFKENADYNAALNISNPKLKSTKEEP

SEQ ID NO: 730 - protein, 726 aa, synthetic construct
SEVEFSHEYWMRHALTLAKRARDEREVPVGAVLVLNNRVIGEGWNRAIGLNDPTAHAEIMALRQGGLVMQNYRLIDATLYVTFEPCVMCAGAMIHSRIGRVVFGVRNNKHGAAGSLMNVLNYPGMNHRVEITEGILADECAALLCDFYRMPRQVFNARKKAQSSINPGGSSGGSGGSETPGTSESATPENSGGSSGSSAKNTITKTLKLRIVRPYNSAEVEKIVADEKNNREKIALEKNKGKVKEACSKHLKVAAYCTTQVERNACLFCKARKLDDKFYQKLRGQFPDAVFWQEIGEIFRQLQKQAAEIYNQSLIELYYEIFIKGKGFANASSVEHYLSDVCYTRAAELFKNAAIASGLRGKVKSNFRLKELKNMKSGLPTTKSDNFPIPLVKQKGGQYTGFEISNHNDDFIIKIPFGRWQVKEEIDKYRPWEKFDFEQVRKNPKPISLLLSTQRRKGNKGWSKDEGTEAEIRKVMNGDYQTSYIEVKRGSKIGEKSAWMLNLSIDVPKIDKGVDPSIIGGIDVGVKSPLVCAINNAFSRYSISDNDLFRFNKKVFARRRILLKKNRHKRAGHGTKNKLKPIAILTEKSGRFRKKLIERWACEIANFFIKNKVGTVQMENLESMKRKEDNYFNIRLRGFWPYAEMQNKIEFKLKQYGIKIRKVAPNNTSKTCSKCGHLNNHFSFEYRKKNKFPHFKCEKCNFKEDADYNAALNISNPKLKSTKEEP

SEQ ID NO: 731 - protein, 726 aa, synthetic construct
SEVEFSHEYWMRRALTLAKRARDEREVPVGAVLVLNNRVIGEGWNRAIGLHDPTAHAEIMALRQGGLVMQNYRLTDATLYVTFEPCVMCAGAMIHSRIGRVVFGVRNSKRGAAGSLMNVLNYPGMNHCVEITEGILVDECAALLCDFYRMPRQVLNAQKKAQSSISSGGSSGGSSCSETPGASESVTPKSSGGSSGGSAKNTITKTLKLRIVRPYNSAEVEKIVADEKNNREKIALEKNKDKVKEACSKHLKVASYCTTQVERNACLFCKARRLDDKFYQKLRGQFPDAVFWQELGEIFRQLQKQAAEIYNQSLIELYYEIFIKGKGFANASSVEHYLSDVCYTRAAELFKNAAIASGLRGKVKSNFRLKELKNMKSGLPTTKSDNFPIPLVKQKGGQYTGFEISSHNDDFIIKIPFGRWQVRKEIDKYRPWEKFDFEQVRKSPKPISLLLSTQRRKRNKGWSKDEGTEAEIRKVMNGDYQTSYIEVKRGSKTGEKSAWMLNLSIDVPKVDKGVDPSIIGGIDVGVKSPLVCAINNAFSRYSISDNDLFRFNKKMFARRRILLKKNRHKRAGHGAKNKLKPISILTEKSKRFRKKLIERWACEIADFFIKNKVGTVQMENLESMKKKEDSYFNIRLRGFWPYAEMQNRIEFKLKQYGIEIRKVAPNNTSKTCSKCGHLNNYFNFEYRKMNKFPHFKCKKCNFKENADYNAALNISNPKLKSTKEKP

SEQ ID NO: 732 - protein, 726 aa, synthetic construct
SEVEFSHEYWMRHALTLAKRARDEREVPVGAVLVLNNRVIGEGWNRAIGLHDPTAHAEIMALRQGGLVMQNYRLTDATLYVTFEPCVMCAGAMIHSRIGRVVFGVRNSKRGAAGSLMNVLNYPGINHCVEITEGILVDECAALLCDFYRMPRQVLNAQKKAQSSISSGGSSGGSSGSETPGASESVTPKSSVGSSAGPTKNTITKTLKLRIVRPYNSAEVEKIVADEKNNREKTALEKNKDKVEEACSKHLKVATYCTTQVERNACLFCKARKLDDKFYQKLRGQFPDAVFWQEISEIFRQLQKQAAEIYNQSLIELYYEIFIKGKGFANASSVEHYLSNVCYTRAAELFKNAAIASGLRGKVKSNFRLKELKNMRSGLPTTKSDNFPIPLVKQKGGQYTGFEISSHNDDFIIKIPFGRWQVKKEIDRFRPWEKFDFEQVRKSPKPISLLLSTQRRKRNKGWSKDEGTEAEIRKVMNGDYQTSYIEVKRGSKTGEKSAWMLNLSIDVPKIDKGVDPSIIGGIDVGVKSPLVCAINNAFSRYSISDNDLFRFNKKMFARRRILLKKNRHKRAGHGAKNKLKPISILTGKSERFRKKLIERWACEIADFFIKNKVGTVQMENLESIKRKEDSYFNIRLRGFWPYAEMQNKIEFKLKQYGIEIRKVAPNNTSKTCSKCGHLNNYFNFEYRKKNKFPHFKCEKCNFKENADYNAALNISNPKLKSTKEGP

SEQ ID NO: 733 - protein, 726 aa, synthetic construct
SEVEFSHEYWMRHALTLAKRARDEREVPVGAILVLNNRVIGEGWNRAIGLHDPTAHAEIMALRQGGLVMQNYRLIDATLYVTFEPCVMCAGAMIHSRIGRVVFGVRNSKHGAAGSLVNVLNYPGMNHRVEITEGVLADECAALLCNFYRMPRQVFNVRKKAQSSINPGGSSGGSSGSETPGTSESATPESSGGSSGGSAKNTITKTLKLRIVRPYNSAEVEKIVADEKNNREKIALEKNKDKVKEACSKHLKVATYCTTQVERNACLFCKARKLDDKFYQKLRGQFPDAVFWQELGEILRQLQKQAAEIYNQSLIELYYEIFIKGRGFANASSVEHYLSDVCYTRAAELFKNAAIASGLRGKVKGNFRLKELKNMKSGLPTTKSDNFPIPLVKQKGGQYTGFEISSHNDDFIIKIPFGRWQVKKEIDKYRPWEKFDFEQVRKSPKPISLLLSTQRRKRNKGWSKDEGTEAEIRKVMNGDYQTSYIEVKRGSKIGEKSAWMLNLSIDVPKIDKGVDPSIIGGIDVGVKSPLVCAINNALSRYSISDKDLFHFNKKMFARRRILLKKNRHKRAGHGAKNKLKPISILTEKSERFRKKLIERWACEVADFFIKNKVGTVQMENLESMKRREDSYFNIRLRGFWPYAKMQSKIEFKLKQYGIEIRKVAPNNTSKTCSKCGHLNNYFNFEYRKKNKFPHFKCEKCNFKENADYNAALNISNPKLKSTKGEP

SEQ ID NO: 734 - protein, 726 aa, synthetic construct
SEVEFSHEYWMRHALTLAKRARDEREVPVGAVLVLNNRVIGVGWNRAIGLHDPTAHAEIMALRQGGLVMQNYRLTDATLYVTFEPCVMCAGAMVHSRIGRVVFGVRNSKRGAAGSLMNVLNYPGMSHCVEITEGILVDECAALLCDFYRMPRQVLNAQKKAQSSISSGGSSGGSGGGETPGASESVTPKNSGGSSGGSAKNTITKTLKLRIVRPYNSTEVEKIVADEKNNREKIALEKNKDKVKEACSKHLKVASYCTTQVERNACLFCKARKLDDKFYQKLRGQFPDAVFWQELGEILRQLQKQAAEIYNQSLIELYYEIFIKGKGFANASSVEHYLSDVCYTRAAELFKNAAIASGLRGKVKGNFRLKELKNMKSGLPTTKSDNFPIPLVKQKGGQYTGFEISSHNDDFIIKIPFGRWQAKKEIDKYRPWEKFDFEQVRKSPKPISLLLSTQRRKRNKGWSKDEGTEAEIRKVMNGDYQTSYIEVKRGSKIGEKSAWMLNLSIDVPKIDKGVDPSIIGGIDVGVKSPLVCAINNALSRYSISDNDLFHFNKKMFARRRILLRKNRHKRAGHGARNKLKPISILTGKSERFRKKLIERWACEIADFFIKNKVGTVQMENLESMKRKEDSYFNIRLRGFWPYAEMQNKIEFKLKQYGIEIRKVAPNNTSKTCSKCGHLNNYFNFEYRKKNKFPHFKCEKCNFKENADYNAALNISNPRLKSTKEEP

SEQ ID NO: 735 - protein, 726 aa, synthetic construct
SEVEFSHEYWMRHALTLAKRARDEREVPVGAILVLNNRVIGEGWNRAIGLHDPTAHAEIMALRQGGLVMQNYRLIDATLYVTFEPCVMCAGAMVHSRIGRVVFGVRNSKRGAAGSLMNVLDYPGMGHRVEITEGILADECAALLCDFYCMPRQVFNAQKRAQSSINSGGSSGGSSGSDTPGTSESATPESSGGGSSGSAKNTITKTLQLRIVRPYNSAEVEKIVADEKNNREKIALEKNKDKVKEACSKHLKVASYCTTQVERNACPFCKARKLDDKFYQRLRGQFPDAVFWQELGEILRQLQKQAAEIYNQSLIELYYEIFIKGRGFANASSVEHYLSDVCYTRAAELFKNAAIASGLRGKVKSNFRLKELKNMKSGLPTTKSDNFPIPLVKQKGGQYTGFEISSHNDDFIIKIPFGRWQVKKEIDKYRPWEKFDFEQVRKSPKPISLLLSTQRRKRNKGWSKDEGTEAEIRKVMNGDYRTSYIEVKRGSKTGERSAWMLNLSIDVPKIDKGVDPSIIGGIDVGVKSPLVCAVNNAFSRYSISDNELFHFNKKMFARRRILLKKNGHKRAGHGAKNKLKPISTLTEKSKRFRKKLIERWACEIADFFIKNKVGTVQMENLESMKRKEDSYFNIRLRGFWPYAEMQNKIEFKLKQYGIEIRKVAPNNTSKTCSKCGHLNDYFNFEYRKKNKFPHFKCEKCNFKENADYNAALNISNPMLKSTKEEP

SEQ ID NO: 736 - protein, 726 aa, synthetic construct
SEVEFSHEYWMRHALTLAKRARDEREVPVGAVLVLNNRVIGEGWNRAIGLHDPTAHAEIMALRQGGLAMQNYRLVDATLYVTFEPCVLCAGAMVHSRIGRVVFGVRNSKRGAAGSLMNVLNHPGMNHRVEITGGILADECAALLCDFYRMPRQVFNAQKKARSNINSGGSSGGSSGSETPGTSESATPESSGGSSGGSAKNTITKTLKLRIVRPYNSAEVEKIVADEKDNREKIALEKNKDKVKEACSKHLKVAAYCTTQVERNACLFCKARKLDDKFYQKLRGQFPDAVFWQEIGEIFRQLQKQAAEIYNQSLIELYYEIFIKGKGFANASSVEHYLSDVCYTRAAELFKNAAIASGLRGKVKSNLRLKELKNMKSGLPTTKSDNFPIPLVKQKGGQYTGFEISSHNDDFIIKIPFGRWQVKKEIDKYRPWEKFDFEQVRKSPKPISLLLSTQRRKRNKGWSKDEGTEAEIRKVMNGDYQTSYIEVKRGSKTGEKSAWMLNLSIDVPKIDKGVDPSIIGGIDVGVKSPLVCAISNAFSRYSISDNDLFRFNKKMFARRRILLKKNRHKRAGHGAKNKLKPISILTGKSERFRKKLIERWACEIADFFIKNKVGTVQMENLESMKRKEDSYFNIRLRGFWPYAEMQNKIEFKLKQYGIEIRKVAPNNTSKTCSKCGHLNNYFSFEYRKKNKFPHFKCEKCNFKENADYNAALNISNPKLKSTKEEP

SEQ ID NO: 737 - protein, 726 aa, synthetic construct
SEVEFSHEHWMRHALTLAKRARDEREVPVGAVLVLNNRVIGEGWNRTIGLHDPTAHAEIMALRQGGLVMQNYRLTDATLYVTFEPCVMCAGAMIHSRIGRVVFGVRNSKRGAAGSLMNVLNYPGMNHCVEITEGILVDECAALLCDFYRMPRQVLNAQKKAQSSTSSGGSSGGSSGSETPGASGSVTPKSSGGSSAGSTKDTITKTLKLRIVRPYNSAEVEKIVADEKNSREKIALEKNKDKVKEACSEHLKVASYCTTQVERNACPFCKARKLDDKFYQKLRGQFPDAVFWQELGGILRQLQKQAAEIYNQSLIELYYEIFIKGRGFANASSVEHYLSDVCYTRAAELFKNAAIASGLRGKVKSNFRLKELKNMKSSLPTTKSDNFPIPLVKQKGGQYTGFEISSHNDDFIIKIPFGRWQVKKEINKHRPWEKFDFEQVRKSPKPISLLLSTQRRKRNKGWSKDEGTEAEIRKVMNGDYQTSYIEVKRGSKIGEKSAWMLSLSIDVPKIDKGVDPSIIGGIDVGVRSPLVCAIDNAFSRYSISDNDLFHFNKKMFARRRILLKKNRHKRAGHGAKNKLKPISILTEKSKRFRKKLIERWACEIADFFIKNKVGTVQMENLESMKRKEDSYFNIRLRGLWPYAEMQNKIEFKLKQYGIEIRKVAPNNTSKTCSKCGHLNNYFNFEYRKKNKFPHFKCEKCNFKEDADYNAALNISNPKLKSTKEEP

SEQ ID NO: 738 - protein, 726 aa, synthetic construct
SEVEFSHEYWMRHALTLAKRARDEREVPVGAILVLNNRVIGEGWNRAIGLHDPTAHAEIMALRQGGLVMQNYRLIDATLYVTFEPCVMCAGAMIHSRIGRVVFGVRNSKHGAAGSLVNVLNYPGMNHRVEITEGILADECAALLCDFYRMPRQVFNARKKAQSSINPSGSSGGSSGSVTPGTSESATPESSGGGFGGSAKNTITKTLQLRIVRPYNSAEVEKIVADEKNNREKIALEKNKGKVKEACSKHLKVAAYCTTQVERNACLFCKARRLDDKFYQKLRGQFPDAVFWQEIGEIFRQLQKQAAEIYNQSLVELYYEILIKGKGIANASSVEHYLSDVCYTRAAELFKNAAIASGLRNKIKSNFRLKELRNMKSGLPTTKSDNFPIPLVRQKGGQYTGFEISNHNGDFIIKIPFGRWQVKKEIDKYRPWEKFDFEQVRKSPKPISLLLSTQRRKRNKGWSKDEGTEAEIRKVMNGDYQTSYIEVKRGSKIGEKSAWMLNLSIDVPKIDKGVDPSIIGGIDVGVKSPLVCAISNAFSRYSISDNDLFHFNKKMFARRRILLGKNRHKRAGHGVKNKLKPITILTEKSGRFRKKLIERWACEIADFFVKNKVGTVQMENLESMKRKEDSYFNIRLRGFWPYAEMQNKIEFKLKQYGIKVRKVAPNNTSKTCSKCGHLNNYFSFEYRKKNKFPHFKCEKCNFKENADYNAALNISNPKLKSTKEEP

SEQ ID NO: 739 - protein, 726 aa, synthetic construct
SEVEFSHEYWMRHALTLAKRARDEREVPVGAVLVLNNRVIGEGWNRAIGLHDPTAHAEIMALRQGGLVMQNYRLTDATLYVTFEPCVMCAGAMIHSRIGRVVFGVRNSKHGAAGSLVNVLNYPGMNHRVEITEGILADECAALLCDFYRMPRRVFNARKKAQSSIDPGGPSDGSSGSETPGISESATPESSGGSSGGSAKNTITKTLKLRIVRPYNSTEVEKIVADEKNSREKIALEKNKDKVKEACSKHLKVASYCTTQVERNACLFCKARKLDDKFYQKLRGQFPDAVFWQELGEIFRQLQKQAAEIYNQSLIELYYEIFIKGKGFANASSVEHYLSDVCYTRAAELFKNAAIASGLRGKVKSNFRLKELKNMKSGLPTTKSDNFPIPLVKQKGGQYTGFEISSHNDDFIIKIPFGRWQVKKEIDKYRPWEKFDFEQVRKSPKPISLLLSIQRRKRSKGWSKDEGTEAEIRKVMNGDYQTSYIEVKRGSKIGEKSAWMLNLSIDVPKIDKGVDPSIIGGIDVGVKSPLVCAVNNAFSRYSISDNELFHFNKKMFARRRILLKKNRHKRAGHGAKNKLKPISTLTERSKRFRKKLIERWACEIADFFIKNKVGTVQMENLESMKRKEDSYFNIRLRGFWPYAEMQNKIEFKLKQYGIEIRKVAPNNTSKTCSKCGHLNNYFNFEYRKKNKFPHFKCERCNFKEDADYNAALNISNPKLKSTKGES

SEQ ID NO: 740 - protein, 726 aa, synthetic construct
GEVELSHEYWMRHALTLAKRARDEREVPVGAVLVLNNRVIGEGWNRAIGLHDPTAHAEIMALRQGGLVMQNYRLIDATLYVTFEPCVMCAGAMVHSRIGRVVFGVRNSKRGAAGSLMNVLDYPGMGHRVEITEGILADECAALLCDFYCMSRQVFNAQKRAQSSINSGGSSDGSSGGETPGTSESATPESSGGSPGGSAKNTITKTLKLRIVRPYNSAEVEKIVADEKNNREKIALEKNKDKVKEACSKHLKVAAYCTTQVERNACLFCKARKLDDKFYQKLRGQFPDAVFWQEIGEVFRQLQKQAAEVYNQSLIELYYEIFIKGKGFANASSVEHYLSDVCYTRAAELFKNAAIASGLRGKVKSNFRLKELKNMRSGLPTTKSDNFPIPLVKQKGGQYTGFEISSHNDDFIIKIPFGRWQVKKEINKFRPWEKFDFEQVRRSPKPISLLLSTQRRKKNKGWSKDEGTEAEIRKVMNGDYQTSYIEVKRGSKIGEKSAWMLNLSIDVPKIDKGVDPSIIGGIDVGVKSPLVCAINNAFGRYSISDNDLFHFNKKMFARRRILLKKNRHKRAGHGAKNKLKPITILTEKSKRFRKKLIERWACEIADFFIKNKVGTVQMENLESMKRKEDSYFNIRLRGFWPYAEMQNKIEFKLKQYGIKVRKVAPNNTSKTCSKCGHLNNYFSFEYRKKNKFPHFKCEKCNFKENADYNAALNISNPKLKSTKEEP

SEQ ID NO: 741 - protein, 726 aa, synthetic construct
SEVEYSHEYWMRHALTLAKRARDEREVPVGAILVLNNRVIGEGWNRAIGLHDPTAHAEIMALRQGGLVMQNYRLIDATLYVTFEPCVMCAGAMIHSRIGRVVFGVRNNKHGAAGSLVNVLNYPGMNHRVEITEGILADECAALLCDFYRMPRQVFNARKKAQSSISPGGSSGGSSGSETPGTSESPTPESSGGSPGGSAKNTITKTLKLRIVRPYNSAEVEKIVADEKDNREKIALEKNKDKVKEACSKHLKVAAYCTTQVERNACLFCKARKLDDKFYQKLRGQFPDAVFWQEIGEIFRQLQKQAAEIYNQSLIELYYEIFIKGKGFANASSVEHYLSDVCYTRAAELFKNAAIASGLRGKVKSNFRLKELKNMKSGLPTTKSDNFPIPLVKQKGGQYTGFEISSHNDDFIIKIPFGRWQVKEEIDKYRPWEKFDFEQVRKNPKPISLLLSTQRRKRNKGWSKDEGTEAEIRKVMNGDYQTSYIEVKRGSKIGEKSAWMLNLSIDVPKIDKGVDPSIIGGIDVGVKSPLVCAINNAFSRYSISDNDLFRFNKKMFARRRILLKKNRHKRAGHGAKNKLKPITILTEKSRRFRKKLIERWACEIADFFIKNKVGTVQMESLESMKRKEDSYFNIRLRGFWPYAEMQNKIEFKLKQYGIKIRKVAPNNTSKTCSKCGHLNNYFSFEYRKKNKFPHFKCEKCNFKESADYNAALNISNPKLMSTKEEP

SEQ ID NO: 742 - protein, 726 aa, synthetic construct
SEVEFSHEYWMRHALTLAKRARDEREVPVGAILVLNNRVIGEGWNRAIGLHDPTAHAEIMALRQGGLVMQNYRLIDATLYVTFEPCVMCAGAMIHSRIGRVVFGVRNNKHGAAGSLVNVLNYPGMNHRVEITEGILADECAALLCDFYRMPRQVFNARKKAQSNINSGSSSGGSSGSETPGTSESATPVSSSGSSGGSAKNTITKTLKLRIVRPYNSAEVEKIVADEKNNREKIALAKNKDKVKEACSEHLKVAAYCTTQVERNACLFCKARKLDDKFYQKLRGQFPDAVFWQEIGEIFRQLQKQAAEIYNQSLVELYYEIFIKGKGFANASSVEHYLSDVCYTRAAELFKNAAIASGLRGKVKSNFRLKELKNMKSGLPTTKSDNFPIPLVKQKGGQYTGFEISNHNGDFIIKIPFGRWQVKKEINKYRPWEKFDFEQVRKSPKPISLLLSTQRRKRNKGWSKDEGTEAEIRKVMNGDYQTSYIEVKRGSKIGEKGAWMLNLSIDVPKIDKGVDPSIIGGIDVGVKSPLVCAINNALSRYSISDNDLFHFNKKMFARRRILLKKNGHKRAGHGARNKLKPIAVLTEKSKRFRKKLIERWACEIANFFIKNKVGTVQMENLESMKRKEDSYFNIRLRGFWPYAEMQNMIEFKLRQYGIEIRKVAPNNTSKTCSKCGHLNNYFNFEYRKKNKFPYFKCAKCNFKENADYNAALNISNPKLKSTKEEP

SEQ ID NO: 743 - protein, 726 aa, synthetic construct
SEVEFSHEYWMRHALTLAKRARDEREVPVGAILVLNNRVIGEGWNRAIGLHDPTAHAEIMALRQGGLVMQNYRLIDATLYVTFEPCVMCAGAMIHSRIGRVVFGVRNSKHGAAGSLVNVLNYPGMNHRVEITEGILADECAALLCDYYRMPRQVFNARKKAQSSINSGGSSDGGSGSETPGTSESATPESSGGSSGGSAKNTITKTLKLRIVRPYNSAEVEKIVADEKNNREQIALEKNKGKVKEACSKHLKVASYCTTQVERNACLFCKARKLDDKFYQKLRGQFPDAVFWQELGGIFRQLQKQAAEIYNQSLIELYYEIFIKGKGITNASRVEHYLSDVCYTRAAELFKNAAIASGLRNKIKSNFRLKELRNMKSGLPTTKSDNFPIPLVKQKGGQYTGFEIGNHNGDFIIKIPFGRWQVKKEIDKYRPWEKFDFEQVRKSPKPISLLLSIQRRKRNKGWSKDEGTEAEIRKVMSGDYQTSYIEVKRGSKIGEKSAWMLNLSIDVPKIDKGVDPSIIGGIDVGVKSPLVCAINNALSRYSISDNDLFHFNKKMFARRRILLRKNRHKRAGHGARNKLKPITVLTEKSERFRRKLIERWACEIANFFIKNKVGTVQMENLESMKRREDSYFNIRLRGFWPYAEMQNKIEFKLKQYGIEIRKVAPNNTSRTCSKCGHLNNYFNFEFRKKNKFPHFKCEKCNFKENADYNAALNISNPKLKSTKEEP

SEQ ID NO: 744 - protein, 726 aa, synthetic construct
SEVEFSHEYWMRHALTLAKRARDEREVPVGAVLVLNNRVIGEGWNRTTGLHDPTAHAEIMALRQGGLVMQNHRLVDATLYVTFEPCVMCAGAMIHSRIGRVVFGVRNSKRGAAGSLTNVLNYPGMNHRVEITEGILVDECAALLCDFYRMPRHVLNAQKKAQSSISSGGSSGGCSGSEMPGASESVTPKSSGGSSAGSTKNTITKTLKLRIVRPYNSAEVEKIVADEKNSREKIALERNKDKVKEACSEHLKVAAYCTTQVERNACLFCKARKLDDKFYQKLRGQFPDAVFWQEIGEIFRQLQKQAAEIYNQSLIELYYEIFIKGKGFANASSVEHYLSDVCYTRAAELFKNAAIASGLRGKVKSNFRLKELKNMKSGLPTTKSDNFPIPLVKQKGGQYTGFEISSHNDDFIIKIPFGRWQVKREIDKYRPWERFDFEQVRKSPKPISLLLSTQRRKRNKGWSKDEGTEAEIRKVMNGDYQTSYIEVKRGSKIGEKSAWMLNLSIDVPKIDKGVDPSIIGGIDVGVKSPLVCAINNAFSRYSISDNDLFHFNKKMFARRRILLKKNRHKRAGHGAKNKLKPITILTEKSRRFRKKLIERWACEIADFFIKNKVGTVQMENLESMKRKEDSYFNIRLRGFWPYAEMQNKIEFKLRQYGIEVRKVAPNNTSKTCSRCGHLNNYFNFEYRKKNKFPHFKCEKCNFKENADYNAALNISNPKLKGTKEEP

SEQ ID NO: 745 - protein, 726 aa, synthetic construct
SEVEYSHEYWMRHALTLAKRARDEREVPVGAILVLNNRVIGEGWNRAIGLHDPTAHAEIMALRQGGLVMQNYRLIDATLYVTFEPCIMCAGAMIHSRIGRVVFGVRNNKHGAAGSLMNVLSYPGMNHRVEITEGILADECAALLCDFYRMPRRVFNAQKKAQSSINSGGSSGGGSSSDTPSTSESTTPESSGGSSGGPAKNTITKTLKLRIVRPYNSAEVEKIVADEKNNREKTALEKNKDKVKEACSKHLKVAAYCTTQVERNACLFCKARKLDDKFYQKLRGQFPDAVFWQEVGEIFRQLQKQAAEIYNQSLIELYYEIFIKGKGFANASSVEHYLSDVCYTRAAELFKNAAIASGLRNKIKSNFRLKELRNMKSGLPTTKSDNFPIPLVRQKGGQYTGFEISNHDGDFIIKIPFGRWQVKKEICKYRPWEKFDFEQVRKSPKPISLLLSTQRRKRNKGWGKDEGTEAEIRKVMNGDYRTSYIEVKRGSKTGEKSAWMLSLSIDVPKIDKGVDPSIIGGIDVGVKSPLVCAINNAFSRYSISDNDLFRFNKKMFARRRILLKKNRHKRAGHGAKNKLKPISILTGKSERFRKKLIERWACEIADFFIKNKVGTVQMENLESMKRKEDSYFNIRLRGFWPYAEMQNKIEFKLKQYGIEIRKVAPNNTSKTCSKCGHLNNYFNFEYRKKNKFPHFKCEKCNFKENADYNAALNISNPKLKSTKEEP

SEQ ID NO: 746 - protein, 726 aa, synthetic construct
SEVEFSHEYWMRHALTLAKRARDEGEVPVGAVLVLNNRVIGEGWNRAIGLHDPTAHAEIMALRQGGLVMQNYRLTDATLYVTFEPCVMCAGAMIHGRIGRVVFGVRNSKRGAAGSLVNVLDYPGMGHRVEITEGILADECAALLCDFYCMPRQVFNAQKRAQSSINSGSSSGGSSGSETPGTSESATPESSGGSSSGSAKNTITKTLQLRIVRPYNSAEVEKIVADEKNNREKIALEKNKDKVKEACSEHLKVAAYCTTQVERNACLFCKARKLDDKFYQKLRGQFPDAVFWQEIGEIFRQLQKQAAEIYNQSLIELYYEIFIKGKGFANASSVEHYLSDVCYTRAAELFKNAAIASGLRGKVKSNFRLKELKNMKSGLPTTKSDNFPIPLVKQKGGQYTGFEISSHDDDFIIKIPFGRWQVKEEIDKYRPWEKFDFEQVRKNPKPISLLLSTQRRKRNRGWSKDEGTEAEIRKVMNGDYQTSYIEVKRGSKIGEKSAWMLNLSIDVPKIDKGVDPSIIGGIDVGVKSPLVCAINNAFSRYSISDNDLFRFNKKMFARRRILLGKNRHKRAGHGAKNKLKPISILTGKSERFRKKLIERWACEIADFFIKNKVGTVQMENLESMKRREDSYFNIRLRGFWPYAEMQNKIEFKLKQYGIEIRKVAPNNTSKTCSKCGHLNNYFNFEYRKKNKFPHFKCEKCNFKENADYNAALNISNPKLKSTKEEP

SEQ ID NO: 747 - protein, 726 aa, synthetic construct
SEVEFSHEYWMRHALTLAKRARDEREVPVGAILVLNNRVIGEGWNRAIGLHDPTAHAEIMALRQGGLVMQNYRLIDATLYVTFEPCVMCAGAMIHSRIGRVVFGVRNNKHGAAGSLVNVLDYPGMNHRVEITEGILADECAALLCDFYRMPRQVFNARKKAQSSISPGGSSGGSSGSETPGAIESVTPKSSGGRSGGSAKNTFTKTLKLRIVRPYNSAEVEKIVADEKNNREKIALEKNKGKVKEACSKHLEVAAYCTTQVERSACLFCKARKLDDKFYQKLRGQFPDAVFWQELGEIFRQLQKQAAEIYNQSLIELYYEIFIKGKGFANASSVEHYLSDVCYTRAAELFKNAAIASGLRGKVKSNFRLKELKNMKSGLPTTKSDNFPIPLVKQKGGQYTGFEISSHNDDFIIKIPFGRWQVKKEIDKYRPWEKFDFEQVRKSPKPISLLLSTQRRKRNKGWSKDEGTEAEIRKVMNGDYQTSYIEVKRGSKTGEKSAWMLNLSIDVPKIDKGVDPSIIGGIDVGVKSPLVCAINNAFSRYSISDNELFHFNKKMFARRRILLKKNRHKRAGHGAKNKLKPISVLTEKSERFRKKLIERWACEIADFFIKNKVGTVQMENLESMKRKEDSYFNIRLRGFWPYAEMQNRIEFKLKQYGIEIRKVAPNNTSKTCSKCGHLNNYFNFEYRKKNKFPHFKCEKCNFKENADYNAALNISNPKLKSTKEEP

SEQ ID NO: 748 - protein, 726 aa, synthetic construct
SEVEFSHEYWMRHALALAKRARDEREVPVGAVLVLNNRVIGEGWNRAIGLHDPTAHAEIMALRQGGLVMQNYRLVDATLYVTFEPCVLCAGAMVHSRIGRVVFGVRNSKRGAAGSLMNVLNYPGMNHRVEITEGILADECAALLCDFYRMPRQVFNAQKKARSNINSGGSSGGSSDSETPGTSESATPESSGGSSGGSAKNTITKTLKLRIVRPYNSAEVEKIVADEKNNREKIALEKNKDKVKEACSKHLKVAAYCTTQVERNACLFCKARKLDDKFYQKLRGQFPDAVFWQEIGEIFRQLQKQAAEIYNQSLIELYYEIFIKGKGFANASSVEHYLSDVCYTRAAELFKNAAIASGLRGKVKSNFRLKELKSMKSGLPTTKSDNFPIPLVKQKGGQYTGFEISSHNDDFIIKIPFGRWQVKKEIDKYRPWEKFDFEQVRKNPKPISLLLSTQRRKRNKGWSKDEGTEAEIRKVMNGDYQTSYIEVKRGSKIGEKSAWMLNLSIDVPKIDKGVDPSIIGGIDVGVKSPLVCAINNAFSRYSISDNDLFRFNKKVFARRRILLKKNRHKRAGHGTKNKLKPITILTEKSGRFRKKLIERWACEIANFFIKNKVGTVQMENLEGMKRKEDSYFNIRLRGFWPYAEMQNKIEFKLKQYGIKIRKVAPNNTSKTCSKCGHLNNYFSFEYRKKNKFPHFKCEKCNFKEDADYNAALNISNPKLKSTKEEP

SEQ ID NO: 749 - protein, 726 aa, synthetic construct
SEDEFSHEYWMRHALTLAKRARDGREVPVGAVLVLNNRVIGEGWNRAIGLHDPTAHAEIMALRQGGLVMQNYRLIDATLYVTFEPCVMCAGAMVHSRIGRVVFGVRNSKRGAAGSLMNVLDYPGMGHRVEITEGILADECAALLCDFYCMPRQVFNAQKRAQSSINSGGSSGGSSGSETPGTSESATPESSGGGSSGSAKNTITKTLQLRIVRPYNSAEVEKIVADEKNNREKIALEKNKGKVKEACSKHLEVAAYCTTQVERNACLFCKARKLDDKFYQKLRGQFPDAVFWQEIGEIFRQLQKQAAEIYNQSLVELYYEIFIKGKGIANASSVEHYLSDVCYTRAAELFKNAAIASGLRNKVKSNFRLKELRNMKSGLPTTKSDNFPIPLVRQKGGQYTGFEISSHDDDFIIKIPFGRWQVKEEIDKYRPWEKFDFEQVRKSPKPISLLLSTQRRKRNKGWSKDEGTEAEIRKVMNGDYQTSYIEVKRGSKTGEKSAWMLNLSIDVPKIDKGVDPSIIGGIDVGVKSPLVCAINNAFSRYSISDNDLFRFNKKMFARRRILLKKNRHKRAGHGAKNKLKPISILTGKSERFRRKLIERWACEIADFFIKNKVGTVQMENLESMKRKEDSYFNIRLRGFWPYAEMQNKIEFKLKQYGIEIRKVAPNNTSKTCSKCGHLNNYFSFEYRKKNKFPHFKCEKCNFKEDADYNAALNISNPKLKSTKEEP

SEQ ID NO: 750 - protein, 726 aa, synthetic construct
SEAEFSHEYWMRHALTLAKRARDEREVPVGAILVLNNRVIGEGWNRAIGLHDPTAHAEIMALRQGGLVMQNYRLIDATLYVTFEPCVMCAGAMIHSRVGRVVFGVRNSKHGAAGSLMNVLNYPGMNHRVEITEGILADECAALLCDFYRMPRRVFNARKEAQSSIDPGGPSGGSSGSETPGTSESATPESSGGSSGGSAKNTITKTLKLRIVRPYNSTEVEKIVADEKNNREKIALEKNKDKVKEACSKHLKVASYCTTQVERNACLFCKARKLDDKFYQKLRDQFPDAVFWQEIGEIFRQLQRQAAEIYNQSLIELYYEIFIKGKGIANASSVEHYLSDVCYTRAAELFKNAAIASGLRNKIKSNFRLKELRNMKSGLPTTKSDNFPIPLVRQKGGQYTGFEISNHNGDFIIKIPFGRWQVKKEISKHRPWEKFDFEQVRKSPKPISLLLSTQRRKRNKGWGKDEGTEAEIRKVMNGDYQTSYIEVKRGSKFGEKSAWMLNLSIDVPKIDKGVDPSIIGGIDVGVKSPLVCAINNAFSRYSISDNDLFRFNKKMFARRRILLGKNRHKRAGHGVKNKLKPITILTEKSGRFRKKLIERWACEIADFFVKNKVGTVQMENLESMKRKEDSYFNIRLRGFWPYAEMQNKIEFKLKQYGIKVRKVAPNNTSKTCSKCGHLNNYFSFEYRKKNKFPHFKCEKCNFKENADYNAALNISNPKLKSTKEEP

SEQ ID NO: 751 - protein, 726 aa, synthetic construct
SEVEFSHEYWMRHALTLAKRARDEREVPVGAVLVLNNRVIGEGWNRAIGLHDPTAHAEIMALRQGGLVMQNYRLVNATLYVTFEPCVMCAGAMIHSRIGRVVFGVRNSRRGAAGSLMNVLDYPGMNHRVEITEGILADECAALLCDFYRMPRQVLIAQKKAQSNINPGSSSGGSSGSETPGTSESATPGSSGGSSGGSAKNTITKTLKLRIVRPYNSAEVEKIVADEKNNREKIALEKNKDKVKEACSEHLKVAAYCTTQVERNACPFCKARKLDDKFYRKLRGQFPDAVFWQEIGEIFRQLQKQAAEIYNQSLIELYYEIFIKGRGFANASSVEHYLSDVCYTRAAELFKNAAIASGLRSKVRSNFRLKELKNMKSGLPTTKSDNFPIPLVKQKGGQYTGFEISSHNSDFIIKIPFGRWQVKEEIDKYRPWEKFDFEQVRKSPKPISLLLSTQRRKRNKGWSKDEGTEAEIRKVMNGDYQTSYIEVKRGSKIGEKSAWMLNLSIDVPKIDKGVDPSIIGGIDVGVKSPLVCAINNAFSRYSISDNDLFRFNKKMFARRRILLGKNRHKRAGHGVKNKLKPITILTEKSGRFRKKLIERWACEIADFFVKNKVGTVQMENLESMKRKEDSYFNIRLRGFWPYAEMQNKIEFKLKQYGIKIRKVAPNNTSKTCSKCGHLNNYFSFEYRKKNKFPHFKCEKCNFKENADYNAALNISNPKLMSTKEVP

SEQ ID NO: 752 - protein, 726 aa, synthetic construct
SEVEFSHEYWMRHALTLAKRARDEREVPVGAVLVLNNRVIGEGWNRAIGLHDPTAHAEIMALRQGGLVMQNYRLVDATLYVTFEPCVLCAGAMVHSRIGRVVFGVRNSKRGAAGSLMNVLNHPGMNHRVEITEGILADECAALLCDFYRMPRQVFNAQKKARSNINSGGSSGGSSGSETPGTSESATPVSSSGSSGGSAKNTITKTLKLRIVRPYNSAEVEKIVADEKDNREKIALEKNKDKVKEACCEHLKVATYCTTQVERNACLFCKARKLDDKFYQKLRGQFPDAVFWQEIGEIFRQLQKQAAEIYNQSLIELYYEIFVKGKGFANASSVEHYLSDVCYTRAAELFKNAAIASGLRGKVKSNFRLKELKNMKSGLPTTKSDNFPIPLVRQKGGQYTGFEISSHNDDFIIKIPFGRWQVKKEIDKYRPWEKFDFEQVRKSPKPISLLLSTQRRKRNKGWSKDEGTEAEIKKVMNGDYQTSYIEVKRGSKIGEKSAWMLNLSIDVPKIDKGVDPSITGGIDVGVKSPLVCAINNALSRYSISDNDLFHFNKKMFARRRILLKKNRHKRAGHGAKNKLKPLTILTGKSKRFRKKLIERWACEIAGFFIKNKVGTVQMENLESMKRREDSYFNIRLRGFWPYAEMQNKIEFKLKQYGIEIRKVAPNNTSKTCSRCGHLNNYFNFEYRKKNKFPHFKCEKCNFKEDADYNAALNISNPKLKSTKEEP

SEQ ID NO: 753 - protein, 726 aa, synthetic construct
SEVEFSHEYWMRHALTLAKRARDEREVPVGAVLVLNNRVIGEGWNRTTGLHDPTAHAEIMALRQGGLVMRNYRLTDATLYVTFEPCVMCAGAMIHSRIGRVVFGVRNSKRGAAGSLMNVLNYPGMNHCVEITEGILVDECAALLCDFYRMPRQVLNAQKKAQSSISPGGSSGGSSGSETPGASGSVTPKSSGGGSSGSAKNTITKTLQLRIVRPYNSAEVEKIVADEKNNREKIALEKNKDKVKEACSKHLKVASYCTTQVERNACPFCKARKLDDKFYQKLRGQFPDAVFWQEVGGIFRQLQKQAAEIYNQSLIELYYEIFIKGKGITNASRVEHYLSDVCYTRAAELFKNAAIASGLRSKVRSNFRLKELKNMKSGLPTTKSDNFPIPLVKQKGGQYTGFEISSHNSDFVIKIPFGRWQVKEEIDKYRPWEKFDFEQVRKSPKPISLLLSTQRRKKNKGWSKDEGTEAEIRRVMNGDYQTSYIEVKRGSKIGEKSAWMLSLSIDVPKIDKGVDPSIIGGIDVGVKSPLVCAINNAFCRYSISDNDLFHFNKKMFARRRILLKKSRHKRAGHGAKNKLKPISILTEKSKRFRKKLIERWACEIADFFIKNKVGTVQMENLESMKRKEDSYFNIRLRGFWPYAEMQNKIEFKLKQYGIEIRKVAPNNTSKTCSKCGHLNNYFNFEYRKKNKFPHFKCEKCSFKENADYNAALNISNPKLKSTREEP

SEQ ID NO: 754 - protein, 726 aa, synthetic construct
SEVEFSHEYWMRHALTLAKRARDEREVPVGAVLVLNNRVIGEGWNRAIGLHDPTAHAEIMALRQGGLVMQNYRLIDATLYVTFEPCVMCAGAMVHSRIGRVVFGVRNSKRGAAGSLMNVLDYPGMGHRVEITEGILADECAALLCDFYCMPRQVFNAQKKAQSSINPGGSSGGSSGSETPGTSESATPESSGGSSGSSAKNTITKALKLRIVRPYNSAEVEKIVADEKNNREKIALEKNKDKVREACSKHLKVAAYCTTQVERNACLFCKARRLDDKFYQKLRGQFPDAVFWQEIGEIFRQLQKQAAEIYNQSLVELYYEIFIKGKGIANASSVEHYLSDVCYTRAAELFKNAAIASGLRNKIKSNFRLKELRNMKSGLPTTKSDNFPIPLVRQKGGQYTGFEISNHNGDFIIKIPFGRWQVKKEISKHRPWEKFDFEQVRKSPKPISLLLSTQRRKRNKGWGKDEGTEAEIRKVMNGDYQTSYIEVKRGSKTGEKSAWMLNLSIDVPKIDKGVDPSIIGGIDVGVKSPLVCAINNAFSRYSISDNDLFRFNKKMFARRRILLKKNRHKRAGHGAKNKLKPISILTGKSERFRKKLIERWACEIADFFIKNKVGTVQMENLESMKRKEDSYFNIRLRGFWPYAEMQNKIEFKLKQYGIEVRKVAPNNTSKTCSKCGHLNNYFSFEYRKKNKFPHFKCEKCNFKENADYNAALNISNPKLKSTKEEP

SEQ ID NO: 755 - protein, 726 aa, synthetic construct
SEVEFSHEYWMRHALTLAKRARDEREVPVGAVLVLNDRVIGEGWNRTTGLHDPTAHAEIMALRQGGLVMQNHRLVDATLYVTFEPCVMCAGAMIHSRIGRVVFGVRNSKRGAAGSLTNVLNYPGMGHRVEITEGILADECAALLCDFYRMPRQVFNAQKKAQSNINPGGSSSGSSGGETPGTSESATPGGSGVSSGGSAKNTITKTLKLRIVRPYNSAEVEKIVADEKNSREKIALEKNKDKVKEACSKHLKMASYCTTQVERNACLFCKARKLDDKFYQKLRGQFPDAVLWQELGEILRQLQKQAAEIYNQSLIELYYEIFIKGRGFANASSVEHYLSDVCYTRAAELFKNAAIASGLRGKVKSNFRLKELKNMKSGLPTTKSDNFPIPLVKQKGGQYTGFEISSHNDDFIIKIPFGRWQVKKEIDKYRPWEKFDFEQVRKSPKPISLLLSTQRRKRNKGWSKDEGTEAEIRKVMNGDYQTSYIEVKRGSKTGEKSAWMLNLSIDVPKIDKGVDPSIIGGIDVGVKSPLVCAINNAFSRYSISDNDLFHFNKKMFARRRILLKKNRRRRAGHGAKNKLKPITILTEKSVRFRKKLIERWACEIADFFIKNKVGTVQMENLESMKRKEDSYFNIRLRGFWPYAEMQNKIEFKLKQYGIEIRRVAPNNTSRTCSKCGHLNNYFSFEYRRKYKFPHFKCEKCNFKEDADYNAALNISNPKLKSTKEEP

SEQ ID NO: 756 - protein, 726 aa, synthetic construct
SEVEFSHEYWMRHALTLAKRARDEREVPVGAILVLNNRVIGVGWNRAIGLHDPTAHAEIMALRQGGLVMQNYRLIDATLYVTFEPCVMCAGAMIHSRIGRVVFGVRNSKHGAAGSLVNVLNYPGMNHRIEITEGILADECAALLCDFYCMPRQVFSARKKAQSSINSGGSSGGSSGSETPGTSESATPKNSGGSSGGSAKNTITKALKLRIVRPYNSAEVEKIVADEKNNRERIALEKNKDKVKEACSKHLKVAAYCTTQVERNACLFCKARKLDDKFYQKLRGQFPDAVFWQELGGIFRQLQKQAAEIYNQSLIELYYEIFIKGKGITNASRVEHYLSDVCYTRAAELFKNAAIASGLRSKVRSNFRLKELKNMKSGLPTTKSDNFPIPLVKQKGGQYTGFEISSHNDDFIIKIPFGRWQVKKEIDKYRPWEKFDFEQVRKSPKPISLLLSTQRRKRNKGWSKDEGTEAEIRKVMNGDYQTSYIEVKRGSKTGEKSAWMLSLSIDVPKIDKGVDPSIIGGIDVGVKSPLVCAINNAFSRYSISDNDLFRFNKKMFARRRILLKKNRHKRAGHGAKNKLKPISVLTEKSGRFRKKLIERWACEIADFFIKNKVGTVQMENLGSMKRKEDSYFNIRLRGFWPYAEMQNKIEFKLKQYGIEIRKVAPDNTSKTCSKCGHLNNYFNFEYRKKNKFPHFKCERCNFKEDADYNAALNISNPKLKSTKEEP

SEQ ID NO: 757 - protein, 726 aa, synthetic construct
SEVEYSHEYWMRHALTLAKRARDEREVPVGAILVLNNRVIGEGWNRAIGQHDPTAHAEIMALRQGGLVMQNYRLIDATLYVTFEPCVMCAGAMIHSRIGRVVFGVRNSKRGAAGSLMNVLNYPGMNHCVEITEGILVDECAALLCDFYRMPRQVLNAQKKAQSSISSGGLSGGSSGSETPGASRSVTPKSSGGSSAGPTKDTITKTLKLRIVRPYNSAEVEKIVTDEKNNREKIALEKNKDKVKEACSKHLKMASYCTTQVERNACLFCKARKLDDKFYQKLRGQFPDAVFWQELGGIFRQLQKQAAEIYNQSLIELYYEIFIKGKGITNASRVEHYLSDVCYTRAAELFKNAAIASGLRSKVRSNFKLKELKSMKSGLPSTKSDNFPIPLVKQKGGQYTGFEISSHDDDFIIKIPFGRWQVKKEIDKYRPWEKFDFEQVRKSPKPISLLLSTQRRKRNKGWSKDEGTEAEIRKVMNGDYQTSYIEVKRGSKIGEKSAWMLNLSIDVPKIDKGVDPGIIGGIDVGVKSPLVCAINNAFSRYSIGDNDLFHYNKKMFARRRILLKKNRHKRAGHGAKNKLKPISILTEKSKRFRKKLIERWACEIADFFIKNKVGTVQMENLESMKRREDSYFNIRLRGFWPYAEMQNKIEFKLKQYGIEIRKVAPNNTSKTCSKCGHLNSYFNFEYRKKNKFPHFKCEKCNFKENADYNAALNISNPKLKSTKEVP

SEQ ID NO: 758 - protein, 726 aa, synthetic construct
SEVEFSHEYWMRHALTLAKRARDEREVPVGAVLVLNNRAIGEGWNRAIGLHDPTAHAEIMALRQGGLVMQNYRLVDATLYVTFEPCVMCAGAMIHSRIGRVVFGVRNNKHGAAGSLMNVLNYPGMNHRVEITEGILADECAALLCDFYRMPRQVFNARKKAQSSINPGGPSGGSSGSKTPGTSESATPESSGGSSGGSAKNTITKTLQLRIVRPYNSAEVEKIVADEKNNREKIALEENKDKVREACSKHLKVASYCTTQVERNACPFCKARKLDDKFYQKLRGQFPDAVFWQELGEILRQLQKQAAEIYNQSLIELYYEIFIKGRGFANASSVEHYLSDVCYTRAAELFKNAAIASGLRGKVKGNFRPKELKNMKSGLPTTKSDNFPIPLVKQKGGQYTGFEISSHNDDFIIKIPFGRWQVKKEIDKYRPWEKFDFEQVRKSPKPISLLLSTQRRKRNKGWSKDEGTEAEIRKVMNGDYQTSYIEVKRGSKTGEKSAWMLNLSIDVPKIDKGVDPSIIGGIDVGVKSPLVCAINNAFSRYSISDNDLFRFNKKMFARRRILLKKNRHQRAGHGAKNKLKPITILTEKSGRFRKKLIERWACEIADFFVKNKVGTVQMENLESMKRKEDSYFNIRLRGFWPYAEMQNKIEFKLKQYGIKVRKVAPNNTSKTCSKCGHLNNYFNFEYRKKNKFPHFKCEKCNFKENADYNAALNISNPKLKSTKEEP

SEQ ID NO: 759 - protein, 726 aa, synthetic construct
SEVEFSHEYWMRHALTLAKRARDGREVPVGAILVLNNRVIGEGWNRAIGLHDPTAHAEIMALRQGGLVMQNYRLTDATLYVTFEPCVMCAGAMIHSRISRVVFGVRNNKHGAAGSLVNVLNYPGMNHRVEITEGILANECAALLCDFYRMPRQVFNARKKAQSSINPSGSSGGSSGSVTPGTSESATPESSGGGSGGSAKNTITKTLQLRIVRPYNSAEVEKIVTDEKNNREKIALEENKDKVKEACSKHLKMAAYCTTQVERNACLFCKARRLDDKFYQKLRGQFPDAVFWQELGEIFRQLQKQAAEIYNQGLIELYYEIFIRGKGTANASSMEHYLSDVCYTRAAELFKNAAIASGLRNKIKSNFRLKELKNMKSGLPTTKSDNFPIPLVKQKGGQYTGFEISNHNGDFIIKIPFGRWQVKKEINKYRPWEKFDFEQVRKSPKPISLLLSTQRRKRNKGWSKDEGTEAEIKKVMNGDYQISYIEVKRGSKIGEKSAWTLNLSVDVPKIDKGVDPSIIGGIDVGVKSPLVCAINNALSRYSISDNDLFHFNKKVFARRRILLKKNRHRRAGHGAKNKLKPITILTEKSKRFRKKLIERWACEIADFFIKNKVGIVQMENLESMKRREDSYFNIRLRGFWPYAEMQNKIEFKLKQYGIGIRKVAPNNTSKTCSRCGHLNNYFNFEHRKKNKFPRFKCEKCNFKENADYNAALNISNPKLKSTKEEP

SEQ ID NO: 760 - protein, 726 aa, synthetic construct
SEVEFSHEYWMRHALTLAKRARDEREVPVGAVLVLNNRVIGEGWNRAIGLHDPTAHAEIMALRQGGLVMQNYRLSDATLYVTFEPCVMCAGAMIHSRIGRVVFGVRNSKRGAAGSLMNVLNYPGMNHCVEITEGILVDECAALLCDFYRMPRQVLSAQKKAQSSISSGGSSGDSSGSETPGASGSVTPKSSVGSSAGSTKNTITKTLKLRIVRPYNSAEVEKIVADEKNNREKIALEKNKDKVKEACSKHLKVAAYCTTQVERNACLFCKARKLDDKFYQKLRGQFPDAVFWQETGEIFRQLQRQAAEIYNQSLIELYYEIFIKGKGFANASSVEHYLSDVCYTRAAELFKNAAIASGLRGKVKSNFRLKELKNMKSGLPTTKSDNFPIPLVKQKGGQYTGFEISSHNDDFIIKIPFGRWQVKKEIDKYRPWEKFVFEQVRKSPKPISLLLSTQRRKRNKGWSKDEGTEAEIRKVMNGDYQTSYIEVKRGSKIGEKSAWMLSLSIDVPKIDKGVDPSIIGGIDVGVKSPLVCAINNAFCRYSISDNDLFHFNKKMFARRRILLKKSRHKRAGHGAKNKLEPISILTEKSKRFRKKLIERWASEIADFFIKNKVGTVQMENLESMKRKEDSYFNIRLRGFWPYAEMQNKIEFKLKQYGIEIRKVAPNNTSKTCSKCGHLNSYFNFEYRKKNKFPHFKCEKCNFKENADYNAALNISNPKLKSTKEEP

SEQ ID NO: 761 - protein, 726 aa, synthetic construct
SEVEFSHEYWMRHALTLAKRARDEREVPVGAVLVLDNRVIGEGWNRAIGLHDPTAHAEIMALRQGGLVMQNYRLIDATLYVTFEPCVMCAGAMIHSRIGRVVFGVRNNKHGAAGSLVNVLNYPGMNHRVEITEGILADECAALLCDFYRMPCQVFNARKKAQSSISPGGSSGGSSGSETPGTSESATPKSSGGSSGGSAKNTITKALKLRIVRPYNSAEVEKIVADEKNNRERIALEKNKDKVKEACSKHLKVAAYCTTQVERNACLFCKARKLDNKFYQKLRGQFPDAVFWQEIGEIFRQLQKQAAEIYNQSLIELYYEIFIKGKGFANASSVEHYLSDVCYTRAAELFKNAAIASGLRGKVKSNFRLKELKNMRSGLPTTKSDNFPIPLVKQKGGQYAGFEISSHNDDFIIKIPFGRWQVKKEIDKYRPWEKFDFEQVRKSPKPISLLLSTRRRKRNKGWSKDEGTEAEIRKVMNGDYQTSYIEVKRGSKIGEKSAWMLNLSIDVPKIDKGVDPSIIGGIDVGVKSPLVCAINNAFSRYSISDNDLFRFNKKVFARRRILLKKNRHKRAGHGTKNKLKPITILTEKSGRFRKKLIERWACEIANFFIKNKVGTVQMENLESMKRKEDSYFNIRLRGFWPYAEMQNKIEFKLKQYGIKIRKVAPNNTSKTCSKCGHLNNYFSFEYRKKNKFPHFKCEKCNFKEDADYNAALNISNPKLKSTKEEP

SEQ ID NO: 762 - protein, 726 aa, synthetic construct
SEVEFSHEYWMRHALTLAKRARDEREVPVGAVLVLNNRVIGVGWNRAIGLHDPTAHAEIMALRQGGLVMQNYRLVDATLYVTFEPCVLCAGAMVHSRIGRVVFGVRNSKRGAAGSLMNVLNYPGMNHRVEITEGILADECAALLCDFYRMPRQVFNAQKKARSNINSGGSSGGGSGSETPSTSKSATPESSGGSSGGSAKNTVTKTLKLRIVRPYNSTEVEKIVADEKNNREKIALEKNKDKVKEACSKHLKVASYCTTQVGRNACLFCKARKLDDKFYQKLRGQFPDAVFWQELGEIFRQLQKQAAEIYNQSLIELYYEIFIKGKGLANASSVEHYLSDVCYTRAAELFKNAAIASGLRGKVKSNFKLKELKSMKSGLPSTKSDNFPIPLVKQKGGQYTGFEISSYNDDLIIKIPFGRWQVKKEIDKYRPWEKFDFEQVRKSPKPISLLLSTQRRKRNKGWSKDEGTEAEIRKVMNGGYQTSYIEVKRGSKTGEKSAWMLNLSIDVPKIDKGVDPSIIGGIDVGVKSPLVCAINNAFSRYSISDNDLFHFNKKMFARRRILLKKNRHKRAGHGAKNKLKPISILTEKSKRFRKKLIERWACEIADFFIKNKVGTVQMENLESMKRKEDSYFNIRLRGLWPYAEMQNKIEFKLKQYGIEVRKVAPNNTSKTCSKCGHLNNYFNFEYRKKNKFPHFKCEKCNFKENADYNAALNISNPKLKSTKEEP

SEQ ID NO: 763 - protein, 726 aa, synthetic construct
SEVEFSHEYWMRHALTLAKRARDEREVPVGAVLVLNNRVIGEGWNRAIGLHDPTAHAEIMALRQGGLVMQNYRLTDATLYVTFEPCVMCAGAMVHSRIGRVVFGVRNSKRGAAGSLMNVLNYPGVNHCVEITEGILVDECAALLCDFYRMPRQVLNAQKKAQSSISSGGSSGGCSGSEMPGASESVTPKSSGGSSGSSAKNTITKTLKLRIVRPYNSAEVEKIVADEKNNREKIALEKNKDKVKEACSRHLKVAAYCTTQVERNACLFCKARRLDDKFYQKLRGQFPDAVFWQEIGEIFRQLQKQAAEVYNQSLVELYYEILIKGKGIANASSVEHYLSDVCYTRAAELFKNAAIASGLRNKIKSNFRLKELRNMKSGLPTTKSDNFPIPLVRQKGGQYTGFEISNYNGDFIIKIPFGRWQVKKEINKHRPWEKFDFEQVRKSPKPISLLLSTQRRKRNKGWSKDEGTEAEIRKAMNGDYQTSYIEVKRGSKIGEKSAWMLSLSIDVPKIDKGVDPRIIGGIDVGVKSPLVCAINNVLSRYSVSDNDLFHFNKKMFARRRILLKKNRHKRAGHGAKNKLKPITTMTEKSKRFRKKLIERWACEIADFFIKNKVGTVQMENLESMKRKEDSYFNIRLRGFWPYAEMQSKIEFKLKQYGIVVRKVAPNNTSKTCSKCGHLNNYFNFEYRKKNKFPHFKCEKCNFKENADYNAALNISNPKLKSTKGEP

SEQ ID NO: 764 - protein, 726 aa, synthetic construct
SEVEFSHEYWMRHALTLAKRARDEREVPVGAVLVLNNRVIGEGWNRTTGLHDPTAHAEIMALRQGGLVMQNHRLVDATLYVTFEPCVMCAGAMIHSRIGRVVFGVRNSKRGAAGSLTNVLNYPGMNHRVEITEGILADECAALLCDFYRMPRQVFGARRKAQSSINSGGSSGGSSGSVTPGTSESATPESSGAGFGDSAKNTITKTLQLRIVRPYNSAEVEKIVADEKNNRERIALEKNKDKVKEACSKHLKVASYCTTQVERNACLFCKARKLDDKFYQKLRGQFPDAVFWQELGEIFRQLQKQAAEIYNQSLIELYYEIFIKGKGLANASSVEHYLSDVCYTRAAELFKNAAIASGLRGKVKSNFRLKELKNMKSGLPTTKSDNFPIPLVKQKGGQYTGFEISSHNDDFIIKIPFGRWQVKKEIVKYRPWEKFDFEQVRKSPKPISLLLSTQRRKRNKGWSKDEGTEAEIRKVMNGDYQTSYIEVKRGSKTGEKSAWMLNLSIDVPKTDKGVDPSIIGGIDVGVKSPLVCAINNSLSRYSICDNDLFRFNKKMFARRRILLKKNRHKRAGHGAKNKLKPITILTKKSGRFRKKLIERWACEIADFFVKNKVGTVQMENLESMKRKEDSYFNIRLRGFWPYAEMQNKIEFKLKQYGIKVRKVAPNNTSKTCSKCGHLNNYFSFEYRKKNKFPHFKCEKCNFKGNADYNAALNISNPKLKSTKEEP

SEQ ID NO: 765 - protein, 726 aa, synthetic construct
SEDEFSHEYWMRHALTLAKRARDEREVPVGAVLVLNNRVIGEGWNRTTGLHDPTAHAEIMALRQGGLVMRNYRLTDATLYVTFEPCVMCAGAMIHSRIGRVVFGVRNSKRGAAGSLMNVLNYPGMNHCVEITEGILVDECAALLCDFYRMPRQVLNAQKKAQSSISPGGSSGGSSGSETPGASESVTPKSSGGSSGGTAKNTITKTLKLRIVRPYNSAEVEKIVADEKNNREKIALEKNKGKVKEACSKHLKVASYCTTQVERNACLFCKARKLDDKFYQKLRGQFPDAVFWQELGEILRQLQKQAAEIYNQSLIELYYEIFIKGKGIANASSVGHYLSDVCYTRAAELFKNAAIASGLRSKIKSNFRLKELRNMRGGLPTTKSDNFPIPLVKQKGGQYTGFEISSHNDDFIIKIPFGKWQVKKEIDKYRPWEKFDFEQVRKSPKPISLLLSTQRRKRNKGWSKDEGTEAEIRKVMNGDYQTSYIEVKRGSKTGEKSAWMLNLSIDVPKIDKGVDPSIIGGIDVGVKSPLVCAINNAFGRYSIGDNDLFHYNKKMFARRRILLKKNRLKRAGHGAKNKLKPISILTEKSKRFRKKLIERWACEIADFFIKNKVGTVQIENLESMKRKEDSYFNIRLRGFWPYAEMQSKIEFKLKQYGIEIRKVAPNNTSKTCSKCGHLNSYFNFEYRKKNKFPHFKCEKCNFKENADYNAALNISNPKLKSTKEEP

SEQ ID NO: 766 - protein, 726 aa, synthetic construct
SEVEFSHEYWMRHALTLAKRARDEREVPVGAILVLNNRVIGEGWNRAIGLHDPTAHAEIMALRQGGLVMQNYRLIDATLYVTFEPCVMCAGAMIHSRIGRVVFGVRNSKHGAAGSLVNVLNYPGMNHRVEITEGILADECAALLCDFYRMPRQVFNARKKAQSSINPSGSSGGSCGSEIPGASESVTPKSSGGSSAGSTKNTITKTLKLRIVRPYNSAEVEKIVADEKNSREKIALERNKDKVKEACSEHLKVAAYCTTQVERNACLFCKARKLDDRFYQKLRGQFPDAVFWQEIGEIFRQLQRQAAEIYNQSLIELYYEIFIKGKGFANASSVEHYLSDVCYTRAAELFKNAAIASGLRGKVKSNFRLKELKNMRSGLPTTKSDNFPIPLVKQKGGQYTGFEISSHNDDFIIKVPFGRWQVKKEINKHRPWEKFDFEQVRKSPKPISLLLSTQRRKRNKGWSKDEGTEAEIRKVMNGDYQTSYIEVKRGSKIGEKSAWMLNLSIDVPKIDKGVDPSIIGGIDVGVKSPLVCAINNALSRYSISDNDLFHFNKKMFARRRILLRKNRHKRAGHGARNKLKPITVLTEKSERFRKKLIERWACEIANFFIKNKVGTVQMENLESMKRKEDSYFNIRLRGLWPYAEMQNKIEFKLKQYGIEVRKVAPNNTSKTCSKCGHLNNYFNFEYRKRNKFPHFKCEKCNFKENADYNAALNISNPKLKGTKEEP

SEQ ID NO: 767 - protein, 726 aa, synthetic construct
SEVEFSHEYWMRHALTLAKRARDEREVPVGAVLVLNNRVIGEGWNRAIGLHDPTAHAEIMALRQGGLVMRNYRLTDATLYVTFEPCVMCAGAMVHSRIGRVVFGVRNSKRGAAGSLMNVLNYPGANHCVEITEGILVDECAALLCDYYRMPRQVLNAQKKAQSSISSGGSSGGCSGSEMPGASESVTPKSSVGSSAGSTKNTITKTLKLRIVRPYNSAEVEKIVADEKDNRERIALEKNKDKVKEACSKHLMVASYCTTQVERSACLFCKARKLDDKFYRELRGQFPDAVFWQEIGEVLRQLQKQAAEIYNQSLIELYYEIFIKGKGFANASSVEHYLSDVCYTRAAELFKNAAIASGLRGKVKSNFRLKELKNMKSGLPTTKSDNFPIPLVKQKGGKYTGFEISSHNDDFIIKIPFGRWQVKKEIDKYRPWEKFDFEQVRKSPKPISLLLSTQRRKRNKGWSKDEGTEAEIRKVMNGDYQTSYIEVKRGSKIGEKSAWMLNLSIDVPKIDKGVDPSIIGGIDVGVKSPLVCAVNNAFSRYSISDNDLFHFNKKMFARRRILLKKNSHKRAGHGAKNKLKPISILTEKSKRFRKKLIERWACEIADFFIKNKVGTVQMENLESMKRKEDSYFNIRLRGFWPYAEMQNKIEFKLKQYGIEIRKVAPNNTSKTCSKCGHLNNYFNFEYRKMNKFPHFKCEKCNFKENADYNAALNISNPKLKSTKEEP

SEQ ID NO: 768 - protein, 726 aa, synthetic construct
SEVEFSHEYWMRRALTLAKRARDEREVPVGAVLVLNNRVIGVGWNRAVGLHDPTAHAEIMALRQGGLVMQNYRLTEATLYVTFEPCIMCAGAMIHSRIGRVVFGVRNSKRGAAGSLMNVLNYPGMNHRVEITEGILADECAALLCDYYRMPRQVFNARKKAQSSINSGGSSDGGSGSETPGTSESATPESSGGSTGGSAKNTITKTLKLRIVRPYNSAEVEKIVADEKNNREKIALEKNKDKVKEACSEHLKVAAYCTTQVERSACLFCKARKLDDKFYQKLRGQFPDAVFWQEIGEIFRQLQKQAAEIYNQSLIELYYEIFIKGKGFANASSVEHYLSDVCYTRAAELFKNAAIASGLRNKTKSNFRLKELRSMKSGLPTTKSDNFPIPLVKQKGGQYTGFEISNHNSDFIIKIPFGRWQAKKEIDKYRPWEKFDFEQVRKSPKPISLLLSTQRRKRNKGWSKDEGTEAEIRRVMNGDYQTSYIEVKRGSKIGEKSAWMLNLSIDVPKIDKGVDPSIIGGIDVGVRSPLVCAINNAFSRYSISDNDLFRFNKKMFARRRILLKKNRHKRAGHGAKNKLRPITILTEKSRRFRKKLIERWACEIADFFIKNKVGTVQMESLESMKRKEDSYFNIRLRGFWPYAEMQNKIEFKLKQYGIEIRKVAPNNTSKTCSKCGHLNNYFNFEYRKKNKFPHFKCEKCNFKENADYNAALNISNPKLKSTKEEP

SEQ ID NO: 769 - protein, 726 aa, synthetic construct
SEVEFSHEYWMRHALTLAKRARDGREVPVGAVLVLNNRVIGEGWNRAIGLHDPTAHAEIMALRQGGLVMQNYRLIDATLYVTFEPCVMCAGAMVHSRIGRVVFGVRNSKRGAAGSLMNVLDYPGMGHRVEITEGILADECAALLCDFYCMPRQVFNAQKRAQSSINSGGSSDGGSGSETPGTSESATPESSGGSSGGSAKNTITKTLKLRIVRPYNSAEVEKIVADEKNNREKTALEKNKDKVKEACSEHLKVAAYCTTQVERSACLFCKARKLDDKFYQKLRGRFPDAVFWQEIGEIFRQLQKQAAEIYNQSLIELYYEIFIKGKGFANASSVEHYLSDVCYTRAAELFKNAAIASGLRGKVKSNFRLKELKNMKSGLPTTKSDNFPIPLVKQKGGQYAGFEISSHNDDFIIKIPFGRWQVKKEIDRYRPWEKFDFEQVRKSPKPISLLLSTQRRKRNKGWSKDEGTEAEIRKVMNGDYQTSYIEVKRGSKTGEKSAWMLNLSIDVPKIDKGVDPSIIGGIDVGVKSPLVCAINNAFSRYSISDNDLFRFNKKMFARRRILLKKNRHKRAGHGAKNKLKPISILTGKSERFRKKLIERWACEIADFFIKNKVGTVQMENLESMKRKEDSYFNIRLRGFWPYAEMQNKIEFKLKQYGVEIRKVAPNNTSKTCSKCGHLNNYFSFEYRKKNKFPHFKCEKCNFKENADYNAALNISNPKLKSTKEGP

SEQ ID NO: 770 - protein, 726 aa, synthetic construct
SEVEFSHEYWMRHALTLAKRARDEREVPVGAVLVLNNRVIGVGWNRAIGLHDPTAHAEIMALRQGGLVMQNYRLTDATLYVTFEPCVMCAGAMVHSRIGRVVFGVRNSKRGAAGSLMNVLNYPGMSHRVEITEGILADECAALLCDFYRMPRQVFNARKKAQSSINSGGSSGGSSGSETPGTSESATPKSSGGSSGGSAKNTITKTLKLRIVRPYNSAEVEKIVADEKNSREKIALEKNKDKVKEACSEHLKVAAYCTTQVERNACLFCKARKLDDKFYQKLRGQFPDAVFWQEIGEIFRQLQKQAAEVYNQSLVELYYEILIKGKGIANASSVEHYLSDVCYTRAAELFKNAAIASGLRGKVKGNFRLKELKNMKSGLPTTKSDNFPIPLVKQKGGQYTGFEISSHNDDFIIKIPFGRWQVKKEIGKYRPWEKFDFEQVRKSPKPISLLLSTQRRKRNKGWSKDEGTEAEIRKVMNGDYQTSYIEVKRGSKTGEKSAWMLNLSIDVPKIDKGVDPSIIGGIDVGVKSPLVCAINNAFSRYSISDNDLFRFNKKMFARRRILLKKNRHKRAGHGAKNKLKPITVLTEKSVRFRKKLIERWACEIADFFIKNKVGTVQMENLESMKRKEDSYFNIRLRGFWPYAEMQNKIEFKLKQYGIEIRKVAPNNTSKTCSKCGHLNNYFNFEYRKKNKFPHFKCEKCNFKENADYNAALNISNPKLKSAKEEP

SEQ ID NO: 771 - protein, 726 aa, synthetic construct
SEVEFSHEYWMRHALTLAKRARDEREVPVGAVLVLNNRVIGEGWNRTTGLHDPTAHAEIMALRQGGLAMQNYRLVDATLYVTFEPCVLCAGAMVHSRIGRVVFGVRNSKRGAAGSLMNVLNYPGMNHRVEITEGILADECAALLCDFYRMPRQVFNARKKARSNINSGGSSGGSSGSETLGTREGATPESSGGGSSGSAKNTITKTLQLRIVRPYNSAEVEKIVADEKNNREKIALEKNKDKVKEACSKHLKVASYCTTQVERSACPFCKARKLDDKFYQKLGGQFPDAVFWQELGEILRQLQKQAAEIYNQSLIELYYEIFIKGRGFANASSVEHYLSDVCYTRAAELFKNAAIASGLRGKVKSNFRLKELKNMKSGLPTTKSDNFPIPLVKQKGGQYTGFEISSHNDDFIIKIPFGRWQVKKEINKYRPWEKFDFEQVRKSPKPISLLLSTQRRKRNKGWGKDEGTEAEIRRVMNGNYQTSYIEVKRGSKIGEKSAWMLNLSIDVPKIDKGVDPSIIGGIDVGVKSPLVCAINNAFSRYSISDNDLFHFNKKMFARRRILLKKNRHKRAGHGAKNKLKRITILTEKSKRFRKKLIERWACEIADFFIKNKVGIVQMENLESMKRKEDSYFNIRLRGFWPYAEMQNRIEFKLKQYGIVVRKVAPNNTSKTCSKCGHLNNYFNFEYRKKNKFPHFKCEKCNFKEDADYNAALNISNPRLKSTKEGP

SEQ ID NO: 772 - protein, 726 aa, synthetic construct
SEVEFSHEYWMRHALTLAKRARDEREVPVGAVLVLNNRVIGEGWNRAIGLHDPTAHAEIMALRQGGLVMQNYRLTDATLYVTFEPCVMCAGAMIHSRIGRVVFGVRNSKRGAAGSLMNVLSYPGMNHCVEITEGILVDECAALLCDFYRMPRQVLNAQKKAQSSISSGGSSGGSSGSETLGASESVAPKSSVGSSASSTKNTITKTLKLRIVRPYNSAEVEKIVADEKDNREKIALEKNKDKVKEACCEHLKVATYCTTQVERNACLFCKARKLDDKFYQKLRGQFPDAVFWQEIGEIFRQLQKQAAEIYNQSLIELYYEIFIKGKGITNASRVEHYLSDVCYTRAAELFKNAAIASGLRSKVRSNFRLKELKNMKSGLPTTKSDNFPIPLVKQKGGQYTGFEISSHNDDFIIKIPFGRWQAKKEIDKYRPWEKFDFEQVRKSPKPISLLLSTQRRKRNKGWSKDEGTEAEIRKVMNGDYQTSYIEVKRGSKTGEKSAWMLNLSIDVPKIDKGVDPSIIGGIDVGVKSPLVCAINNAFSRYSISDNDLFRFNKKMFARRRILLKKNRHKRAGHGAKNKLKPISILTGKGERFRKKLIERWACEIADFFIKNKVGTVQMENLESMKRKEDSYFNIRLRGFWPYAEMQNKIEFKLKQYGIEIRKVAPNNTSKTCSKCGHLNNYFNFEYRKKNKFPHFKCEKCNFKENADYNAALNISNPKLKSTKEEP

SEQ ID NO: 773 - protein, 726 aa, synthetic construct
SEVEFSHEYWMRHALTLAKRARDEREVPVGAVLVLNNRVIGEGWNRAIGLHDPTAHAEIMALRQGGLVMRNYRLTDATLYVTFEPCVMCAGAMIHSRIGRVVFGVRNSKRGAAGSLMNVLNYPGMDHRVEITGGILADECAALLCDFYRMPRRVFNAQKKAQSSINSGGSSGGSSGSVTPGTSESATPESSGGGFGGSAKNTITKTLQLRIVRPYNSAEVEKIVADEKNNREKIALEKNKDKVQEACSKHLKVASYCTTQVERNACLFCKARKLDDKFYQKLRGQFPDAVFWQELGEIFRQLQKQAAEIYNQSLIELYYEIFIKGKGLANASSVEHYLSDVCYTRAAELFKNAAIASGLRGKVKSNFRLKELKNMKSGLPTTKSDNFPIPLVKQKGGQYTGFEISSHNDDFIIKIPFGRWQVKKEIDKYRPWEKFDFEQVRKSPKPISLLLSTQRRKRNKGWSKDEGTEAEIRKVMNGDYQTSYIEVKRGSKIGEKSTWMLNLSIDVPKIDKGVDPNIIGGIDVGVKSPLVCAINNALSRYSISDNDLFRFNKKMFARRRILLKKNRHRRAGHGAKNKLKPISILTEKSKRFRKKLIERWACEIADFFIKNKVGTVQLENLESMKRREDSYFNIRLRGFWPYAEMQNKIEFKLRQYGIEIRKVAPNNTSKTCSKCGHLNNYFDFEYRKKNKFPHFKCEKCNFKENADYNAALNISNPKLRSTKEEP

SEQ ID NO: 774 - protein, 726 aa, synthetic construct
SEVEFSHEYWMRHALTLAKRARDEREVPVGAILVLNNRVIGEGWNRAIGLHDPTAHAEIMALRQGGLVMQNYRLIDATLYVTFEPCVMCAGAMIHSRIGRVVFGVRNSKHGAAGSLVNVLNYPGMNHRVEITEGILADECAALLCDFYRMPRQVFNARKKAQSSINPGGSSGGSSGSEAPGASESATPKSSGGSSGSSTKNTITKTLKLRIVRPYNSAEVEKIVADEKNNREKIALEKNKDKVKEACSEHLKVAAYCTTQVERSACLFCKARKLDDKFYQKLRGQFSDAVFWQEVGEIFRQLQKQAAEIYNQSLIELYYEIFIKGKGFANASSVEHYLSDVCYTRAAELFKNAAIASGLRGKVKSNFRLKELKNMKSGLPTTKSDNFPIPLVKQKGGQYTGFEISSHNDDFIIKIPFGRWQVKKEIDKYRPWEKFDFEQVRKSPKPISLLLSTQRRKRNKGWNKDEGTEAEIRKVMSGDYQTSYIEVKRGSKIGEKSAWMLNLSVDVPKIDKGVDPSIIGGIDVGVKSPLVCAINNAFSRYSISDNDLFHFNKKMFARRRILLKKNGHKRAGHGARNKLKPITIMTEKSKRFRKKLIERWACEIADFFVKNKVGTVQMENLESMKRKEDSYFNIRLRGFWPYAEMQSKIEFKLKQYGIVVRKVTPNNTSKTCSKCGHLNSYFNFEYRKKNKFPHFKCEKCNFKENADYNAALNISNPKLKSTKEEP

SEQ ID NO: 775 - protein, 726 aa, synthetic construct
SEVEFSHEYWMHHALSLAKRARDEREVPVGAVLVLNNRIIGEGWNRAIGLHDPTAHAEIMALRQGGLVMQNYRLTDATLYVTFEPCVMCAGAMVHSRIGRVVFGVRNSKRGAAGSLMNVLNYPGVNHCVEITEGILVDECAALLCDYYRMPRQVFNARKKAQSSTNSGGSSDGGSGSETPGTSESATPKSSGGSSGGSAKNTITKALKLRIVRPYNSAEVEKIVADEKNIREKIALEKNKDKVKEACSKHLKVAAYCTTQVERNACPFCKARKLDDKFYQKLRGQFPDAVFWQELGEILRQLQKQAAEIYNQSLIELYYEIFIKGRGFANTSSVEHYLSDVCYTRAAELFKNAAIASGLRGKVKSNFRLKELKNMKSGLPTTKSDNFPIPLVKQKGGQYTGFEISSHNDDFIIKIPFGRWQVKKEIDKYRPWEKFDFEQVRKSPKPISLLLSTQRRKRNRGWSKDEGTEAEIRKVMNGDYQTSYIEVKRGSKIGEKSAWMLSLSIDVPKIDKGVDPSIIGGIDVGVKSPLVCAINNAYNRYSISDNNLFHFNKKMFARRRILLKKNRHKRAGHGAKNKLKPISILTEKSERFRKKLIERWACEIADFFIRNKVGTVQMENLEGMKRREDSYFNIRLRGFWPYAEMQNKIEFKLKQYGIVVRKVAPNNTSKTCSKCGHLNNYFNFEYRKKNKFPHFKCEKCNFKENADYNAALNISNPKLKSTKEEP

SEQ ID NO: 776 - protein, 726 aa, synthetic construct
SEVEFSHEYWMRHALTLAKRARDEREVPVGAILVLNNRVIGEGWNRANGLHDPTAHAEIMALRQGGLVMQNYRLIDATLYVTFEPCVMCAGAMIHSRIGRVVFGVRNNKHGAAGSLVNVLNYPGMNHRVEITEGILADECAALLCDFYRMPRQVFNARKKAQSSTNPGGSTGGSSGSETPGTSESATPESPGGSSGGSAKNTITKTLKLRIVRPYNSAEVEKIVADEKNNREKIALEKNKDKVKEACSEHLKVAAYCTTQVERSACLFCKARKLDDKFYQKLRGQFPDAVFWQETGEIFRQLQKQAAEIYNQSLIELYYEIFIKGKGFANASSVEHYLSDVCYTRAAELFKNAAIASGLRGKVKSNFRLKELKNMRSGLPTTKSDNFPIPLVKQKGGQYTGFEISSHNDDFIIKIPFGRWQVKKEIDKYRPWEKFDFEQVRKSPKPISLLLSTQRRKRNKGWSKDEGTEAEIRKVMNGDYQTSYIEVKRGSKTGEKSAWMLNLSIDVPKIDKGVDPSIIGGIDVGVKSPLVCAINNAFSRYSISDNDLFRFNKKMFARRRILLRKNRHKRAGHGAKNKLKPISILTGKCERFRKKLIERWACEIADFFIKNKVGTVQMENLESMKRKEDSYFNIRLRGFWPYAEMQNKIEFKLKQYGVEIRKVAPNNTSKTCSKCGHLNNYFNFEYRRKNKFPHFKCERCNFKENADYNAALNISNPKLKSTKEEP

SEQ ID NO: 777 - protein, 726 aa, synthetic construct
SEVEFSHEYWMRHALTLAKRARDEREVPVGAILVLNNRVIGEGWNRAIGLHDPTAHAEIMALRQGGLVMQNYRLTDATLYVTFEPCVMCAGAMIHSRIGRVVFGVRNSKRGAAGSLTNVLNYPGMNHRVEITEGILVDECAALLCDFYRMPRQVFNAQKKAQSTINSGGSSGGSSGSETPGTSESPTPESSGGSPGGSAKNTITKTLKLRIVRPYNSAEVEKIVADEKNNREKIALEKSKDKVKEACSKHLKVAAYCTTQVERNACLFCKARKLDDKFYQKLRGQYPDAVFWQEIGEIFRQLQKQAAEIYNQSLIELYYEIFIKGKGFANASSVEHYLSDVCYTRAAELFKNAAIASGLRGKVKSNFRLKELKNMKSGLPTTKSDNFPIPLVKQKGGQYTGFEISSHNDDFIIKIPFGRWQVKKEIDKYRPWEKFDFEQVRKSPKPISLLLSTQRRKRNKGWSKDEGTEAEIRKVMNGEYQTSYIEVKRGSKIGEKSAWMLSLSIDVPKIDKGVNPSIIGGIDVGVKSPLVCAINNALSRYSVSDNDLFRFNKKMFARRRILLKKNRHKRAGHGAKNKLKPITILTKKSERFRKKLIERWACEIADFFIKNKVGTVQMENLESMKRKEDSYFNIRLRGFWPYAEMQNKIEFKLKQYGIKIRKVAPNNTSKTCSKCGHLNNYFSFEYRKKNKFPHFKCEKCNFKENADYNAALNISNPKLKSTKEEP

SEQ ID NO: 778 - protein, 726 aa, synthetic construct
SEVEFSHEYWMRHALALAKRARDEREVPVGAILVLNNRVIGEGWNRAIGLHDPTAHAEIMALRQGGLVMQNYRLIDATLYVTFEPCVMCAGAMIHSRIGRVVFGVRNSKRGAAGSLMNVLNYPGMNHCVEITEGILVDECAALLCDFYRMPRQVLNAQKKAQSSISPGGSSGGSSGSETPGAGESVTPKSSVGSSAGSTKNTITKTLKLRIVRPYNSAEVEKIVADEKNNREKIALEKNKDKVKEACSKHLKVAAYCTTQVERNACLFCKARKLDDKFYQKLRGQFPDAVFWQEVGEIFRQLQKQAAEIYNRSLIELYYEIFIKGKGFANASSVEHYLSDVCYTRAAELFKNAAIASGLRGKVKSNFRLKELKNMKSGLPTTKSVNFPIPLVKQKGGQYTGFEINSHNDDFIIKIPFGRWQVKKEIDKYRPWEKFDFEQVRKSPKPISLLLSTQRRKRNKGWSKDEGTEAEIRKVMNGDYQTSYIEVKRGSKIGEKSAWMLSLSIDVPKIDRGVDPSIIGGIDVGVKSPLVCAINNALSRYSISDNDLFHFNKKMFARRRILLKKNRHKRAGHGAKNKLKPITILTEKSKRFRKKLIERWACEIADFFVKNKVGTVQMENLESMKRKEDSYFNIRLRGFWPYAEMQNKIEFKLKQYGIEIRKVAPNNTSKTCSKCGHLNNYFNFEYRKKNKFPHFKCEKCNFKENADYNAALNICNPKLKSTKEEP

SEQ ID NO: 779 - protein, 726 aa, synthetic construct
SEVEFSHEYWMRHALTLAKRARDEREVPVGAVLVLNNRVIGEGWNRAIGLHDPTAHAEIMALRQGGLVMQNYRLTDATLYVTFEPCVMCAGAMIHSRIGRVVFGVRNSKRGAAGSLMNVLNYPGMNHRVEITEGILVDECAALLCDFYRMPCQVLNAQKKAQSSISSGGSSGGSSGGDTLGASEGVTPKSSGGGFGGSAKNTITKTLQLRIVRPYNSAEVEKIVADEKNNREKIALEKNKDKVKEACSKHLKVASYCTTQVERNACLFCKARKLDDKFYQKLRGQFPDAVFWQELGEIFRQLQKQAAEIYNQSLIELYYEIFIKGKGFANASSVEHYLSDVCYTRAAELFKNAAIASGLRGKVKSNFRLKELKNMKSGLPTTKSDNFPIPLVKQKGGQYTGFEISSHNDDFIIKIPFGRWQVKEEIDKYRPWEKFDFEQVRKNPKPISLLLSTQRRKRNKGWSKDEGTEAEIRKVMNGDYQTSYIEVKRGSKTGEKSAWMLNLSIDVPKIDKGVDPSIIGGIDVGVKSPLVCAINNAFSRYSISDNDLYRFNKKMFARRRILLKKNRHKRAGHGAKSKLKPISILTGKSERFRKKLIERWACEIADFFIKNKVGTVQMENLESMKRKEDSYFNIRLRGFWPYAEMQNKIEFKLKQYGIKIRKVAPNNTSRTCSKCGHLNNYFSFEYRKKNKFPHFKCEKCNFKEDADYNAALNISNPKLKGTKEEL

SEQ ID NO: 780 - protein, 726 aa, synthetic construct
SEIEFSHEYWMRHALTLAKRARDGREVPVGAVLVLNNRVIGEGWNRAIGLHDPTAHAEIMALRQGGLVMQNYRLIDATLYVTFEPCVMCAGAMIHSRIGRVVFGVRNSKHGAAGSLVNVLNYPGMNHRVEITEGILADECAALLCDFYRMPRQVFNARKRARSNINSGGSSGGSSGSETLGTREGATPESSGGGSGGSAKNTITKTLKLRIVRPYNSAEVEKIVVDEKNNREKVALEKNKDKVKEACSEHLKVAAYCTTQVERSACLFCKARKLDDKFYQKLRGQFPDAVFWQEIGEIFRQLQKQAAEIYNQSLIELYYEIFIKGKGFANASSVEHYLSDVCYTRAAVLFKNAAIASGLRGKVKSNFRLKELKNMKSGLPTTKSDNFPIPLVKQKGGQYTGFEISNHNGDFIIKIPFGRWQVKKEIDRYRPWEKFDFEQVRKSPKPISLLLSTQRRKRNKGWSKDEGTEAEIRKVMNGDYQVSYIEVKRGSKIGEKSAWMLNLSIDVPKIDKGVDPSIIGGIDVGVKSPLVCAINNALSRYSISDNDLFHFNKKMFARRRILLKKNRHKRDGHGARNKLKPITVLAEKSERFRKKLIERWACEIANFFIKNKVGTVQMENLESMKRKEDSYFNIRLRGFWPYAEMQNKIEFKLKQYGIEIRKVAPNNTSKTCSKCGHLNNYFNFEYRKKNKFPHFKCEKCNFKENADYNAALNISNPKLKGTKEEP

SEQ ID NO: 781 - protein, 726 aa, synthetic construct
SEVEFSHEYWMRRALTLAKRARDEREVPVGAVLVLNNRVIGVGWNRAVGLHDPTAHAEIMALRQGGLVMQNYRLIEATLYVTFEPCIMCAGAMIHSRIGRVVFGVRNSKRGAAGSLMNVLNYPGMNHRVEITEGILADECAALLCDYYRMPRQVFNAREKAQSSINSGGSSDGGSGSETPGTSESATPESSGGSSGGSAKNTITKTLKLRIVRPYNSAEVEKIVADEKSNREKIALEKNKDKVKEACSEHLKVAAYCTTQVERSACLFCKARKLDDKFYQKLRGQFPDAVFWQEIGEIFRQLQKQAAEIYNQSLIELYYEIFIKGKGFANASSVEHYLSDVCYTRAAELFKNAAIASGLRGKVKSNFRLKELKNMRSGLPTAKSDNFPIPLVKQKGGQYTGFEISSHNDDFIIKIPFGRWQVKKEFDKYRPWEKFDFEQVRKSPKPISLLLSTQRRKRNKGWSKDEGTEAEIRKVMNGDYQTSYIEVKRGSKTGEKSAWMLNLSIDVPKIDKGVDPSIVGGIDVGVKSPLVCAIDNALSRYSISDNDLFHFNKKMFARRRILLKKNRHRRAGHGAKNKLKPITIMTEKSKRFRKKLIERWACEIADFFIKNKVGTVQMENLESMKRKEDSYFNIRLRGFWPYAEMQNKIEFKLKQYGIVVRKVAPNNTSKTCSQCGHLNNYFNFEYRKKNKFPYFKCEKCNFKENADYNAALNISNPQLKSTKGEP

SEQ ID NO: 782 - protein, 726 aa, synthetic construct
SEVEFSHEYWMRRALTLAKRARDEREVPVGAVLVLNNRVIGVGWNRAVGLHDPTAHAEIMALRQGGLVMQNYRLIEATLYVTFEPCIMCAGAMIHSRIGRVVFGVRNSKRGAAGSLMNVLNYPGMNHRVEITEGILADECAALICDYYRMPRQVFNARKKAQSSINSGGSSDGGSGSETPGTSESATPESSGGSSGGSAKNTITKTLKLRIVRPYNSAEVEKIVADEKNNREKIALEKNKDKVKEACSEHLKVAAYCTTQVERSACLFCKARKLDDKFYQRLRGQFPDAVFWQEIGEIFRQLQKQAAEIYNQSLIELYYEIFIKGKGFANASSVEHYLSDVCYTRAAELFKNAAIASGLRGKVKSNFRLKELKNMRSGLPTTKSDNFPIPLVKQKGGQYTGFEISSHNDDLIIKIPFGRWQVKKEIDKYRPWEKFDFEQVRKSPKPISLLLSTRRRKRNKGWSKDEGTEAEIRKVMNGDYQTSYIEVKRGSKIGEKSAWMLNLSIDVPKIDKGVDPSIIGGIDVGVKSPLVCAINNAFSRYSISDNDLFHFNKKMFARRRILLKKNRHKRAGHGAKNKLKPISILTEKSKRFRKKLIERWACEIADFFIKNKVGTVQMENLESMKRKEDSYFNIRLRGFWPYAEMQNKIEFKLEQYGIEIRKVAPNNTSKTCSKCGHLNNYFNFEYRMKNKFPHFKCEKCNFKENADYNAALNISNPKMKSTKEEP

SEQ ID NO: 783 - protein, 726 aa, synthetic construct
SEVEFSHEYWMRHALTLARRARDEREVPVGAILVLNNRVIGEGWNRAIGLHDPTAHAEIMALRQGGLVMQNYRLTDATLYVTFEPCVMCAGAMVHSRIGRVVFGVRNSKRGAAGSLMNVLSYPGMSHCVEITEGILVDECAALLCDFYRMPRQVLNAQKKAQSSISSGGSSGGSGGGETPGASESVTPKSSGGSSAGSTKNTITKTLKLRIVRPYNSAEVEKIVADEKNNREKIALEKNKDKVKEACSRHLKVASYCTTQVERNACPFCKARKLDDKFYQKLRGQFPDAVFWQEIGEIFRQLQKQAAEIYNQSLIELYYEIFIKGKGTANASSVEHYLSDVCYTRAAELFKNAAIASGLRGKVKSNFRLKELKNMKSGLPTTKSDNFPIPLVKQKGGQYTGFEISSHNDDFIIKIPFGRWQVKKEIDKYRPWEKFDFEQVRKSPKPISLLLSTQRRKRNKGWSKDEGTEAEIRKVMNGDYRTSYIEVKRGSKTGEKSAWMLNLSIDVPKIDKGVDPSIIGGIDVGVKSPLVCAINNAFSRYSISDNDLFRFNKKMFARRRILLKKNRHKRAGHGAKNKLKPISILTGKSERFRKKLIERWACEIADFFIKNKVGTVQIENLESMKRKEDSYFNIRLRGFWPYAEMQSKIEFKLKQYGIEIRKVAPNNTSKTCSKCGHLNNYFDFEYRKKNKFPHFKCEKCNFKENADYNAALNISNPKLKSTKEEP

SEQ ID NO: 784 - protein, 726 aa, synthetic construct
SEVEFSHEYWMRHALTLAKRARDEREVPVGAILVLNNRVIGEGWNRAIGLHDPTAHAEIMALRQGGLVTQNYRLIDATLYVTFEPCVMCAGAMIHSRIGRVVFGVRNSKHGAAGSLMNVLNYPGMNHRVEITEGVLADECAALLSDFYRMPRQVFNAQKKARPYINSGGSSGGSSGSETPGTSESPTPESSGGSSGGSAKNTITKTLKLRIVRPYNSAEVEKIVADEKNNREKIALEKNKDKVKEACSKHLKVASYCTTQVERNACLFCKARKLDDKFYQKLRGQFPDAVFWQETGEIFRQLQRQAAEIYNQSLIELYYEIFIKGKGFANASSVEHYLSDVCYTRAAELFKNAAIASGLRGKVKSNFRLKELKNMKSGLPTTKSDNFPIPLVKQKGGQYTGFEISSHNDDFIIKIPFGRWQVKKEIDKYRPWERFDFEQVRKSPKPISLLLSTQRRKRNKGWSKDEGTEAEIRKVMNGDYQTSYIEVKRGSKIGEKSAWMLNLSIDVPKIDKGVDPSIIGGIDVGVKSPLVCAINNAFSRYSISDNDLFRFNKKMFARRRILLKKNRHKRAGHGAKNKLKPITLLTGKSRRFRKKLIERWACEIADFFIKNKVGTVQMESLESMKRKEDSYFNIRLRGFWPYAEMQNKIEFKLKQYGIKIRKVAPNNTSKTCSKCGHLNNYFNFEYRKKNKFPHFKCEKCNFKENADYNAALNISNPRLKSTKEEP

SEQ ID NO: 785 - protein, 726 aa, synthetic construct
SEVEFSHEYWMRHALTLAKRARDEREVPVGAVLVLNNRVIGEGWNRAIGLHDPTAHAEIMALRQGGLVMQNYRLIDATLYVTFEPCVMCAGAMIHSRIGRVVFGVRNNKHGAAGSLVNVLNYPGMNHRVEITEGILADECAALLCDFYRMPRQVFNARKKAQSSINPGGSSGGSSGSVTPGTSESATPESSGGGFGGSAKNTITKTLQLRIVRPYNSAEVEEIVADEKNNREKIALEKNKDKVKEACSKHLKVASYCTTQVERNACLFCKARKLDDKFYQKLRGQFPDAVFWQELGGIFRQLQKQAAEIYNQSLIELYYEIFIKGKGFANASSVEHYLSDVCYTRAAELFKNAAIASGLRGKVKSNFRLKELKNMKSGLPTTKSDNFPIPLVKQKGGQYTGFEISSHNDDFIIKIPFGRWQVKKEINKYRPWEKFDFEQVRKSPKPISLLLSTQRRKRNKGWSRDEGTEAEIRKVMNGDYQTSHIEVKRGSKTGEKSAWMLNLSIDVPKIDKGVDPSIIGGIDVGVKSPLVCAINNAFSRYSISDNDLFRYNKKMFARRRILLKKNRHKRAGHGAKNKLKPITIMTEKSKRFRKKLIERWACEIADFFIKNKVGTVQMENLESMKRKEDSYFNIRLRGFWPYAEMQNKIEFKLKQYGIVVRKVAPNNTSKTCSKCGHLNNYFNFEYRKRNKFPHFKCEKCNFKENADYNAALNISNPKLKSTKEEP

SEQ ID NO: 786 - protein, 726 aa, synthetic construct
SEVEFSHEYWMRHALTLAKRARDEREVPVGAVLVLNNRAIGEGWNRAIGLHDPTAHAEIMALRQGGLVMQNYRLTDATLYVTFEPCVMCAGAMIHSRIGRVVFGVRNSKRGAAGSLMNVLNYPGMDHRVEITGGILADECAALLCDFYRMPRRVFNAQKKAQSSINSGGSSGGSSGSVTPGTSESATPESSGGSFGGSAKNTITKTLQLRIVRPYNSAEVEKIVADEKNSREKIALEKNKDKVKEACGKHLKVASYCTTQVERNACLFCKARKLDDKFYQKLRGQFPDAVFWQELGEIFRQLQKQAAEIYNQSLIELYYEIFIKGKGLANASSVEHYLSDVCYTRAAELFKNAAIASGLRGKVKSNFKLKELKSMKSGLPSTKSDNFPIPLVKQKGGQYTGFEISSYNDDLIIKIPFGRWQVKKEIDKYRPWEKFDFEQVRKSPKPISLLLSTQRRRRNKGWSKDEGTEAEIRKVMNGDYQTSYIEVKRGSKIGEKSAWMLNLSINVPKIDKGVDPSIIGGIDVGVRSPLVCAINNAFSRYSISDNDLFRFNKKMFARRRILLKKNRHKRAGHGAKNKLKPISILTGKSERFRKKLIERWACEIADFFIKNKVGTVQMENLESMKRKEDSYFNIRLRGFWPYAEMQNKIEFKLKQYGIEIRKVTPNNTSKTCSKCGHLNNYFNFEYRKKNKFPHFKCEKCNFKENADYNAALNISNPKLKSTKEEP

SEQ ID NO: 787 - protein, 726 aa, synthetic construct
SEVEFSHEYWMRHALSLAKRARDEREVPVGAVLVLNNRVIGVGWNRAVGLHDPTAHAEIMALRQGGLVMQNYRLIEATLYVTFEPCIMCAGAMIHSRIGRVVFGVRNSKRGAAGSLMNVLNYPGMNHRVEITEGVLADECAALLCDFYCMPRQVFNAQKRAQSSISSGGSSGGSSGSETPGTSGSVTPKSSVGSSAGSTKNTITKTLKLRIVRPYNSAEVEKIVADEKNNREKIALEKNKGKVKEACSKHLEVAAYCTTQVERNACLFCKARKLDDKFYQKLRGQFPDAVFWQELGEIFRQLQKQAAEIYNQSLIELYYEIFIKGKGFANASSVEHYLSDVCYTRAAELFKNAAIASGLRGKVKSNFRLKELKNMKSGLPTTKSDNFPIPLVKQKGGQYTGFEISSHNDDFIIKIPFGRWQVKKEIDRYRPWEKFDFEQVRKSPKPISLLLSTQRRKRNKGWSKDEGTEAEIRKVMNGDYQTSYVEVKRGSKTGEKSAWMLSLSIDVPKIDKGVDPSIIGGIDVGVKSPLVCAINNAFSRYSISDNDLFRFNKKMFARRRILLKKNRHKRAGHGARNKLKPITVLTEKSKRFRKKLIERWACEIANFFIKNRVGTVQMENLESMKRKEDSYFNIRLRGFWPYAEMQNRIEFKLKQYGIEIRKVAPNNTSKTCSKCGHLNNYFNFEYRKKNKFPHFKCEKCNFKENADYNAALNICNPKLKGTKEEP

SEQ ID NO: 788 - protein, 726 aa, synthetic construct
SEVEFSHEYWMRHALTLARRARDEREVPVGAILVLNNRVIGEGWNRAIGLHDPTAHAEIMALRQGGLVMQNYRLVDATLYVTFEPCVMCAGAMIHSRIGRVVFGVRNNKHGAAGSLMNVLSYPGMNHRVEITEGILADECAALLCDFYRMPRQVFNARKKAQSSINPGGPSGGSSGSKTPGTSESATSEGSGGSSGGSAKDTITKTLKLRIVRPYNSAEVEKIVADEKNSREKIALEKNRDKVKEACSEHLKVAVYCTTQVERNACLFCKARRLDDKFYQKLRGQFPDAVFWQEIGEIFRQLQKQAAEIYNQSLIELYYEIFIKGKGFANASSVEHYLSDVCYTRAAELFKNAAIASGLRGKVKSNFRLKELKNMKSGLPTTKSDNFPIPLVKQKGGQYTGFEISSHNDDFIVKIPFGRWQVKKEIDKYRPWEKFDFEQVRKSPKPISLLLSTQRRKRNKGWSKDEGTEAEIRKVMNGVYQTSYIEVKRGSKIGEKSAWMLNLSIDVPKIDKGVDPRIVGGIDVGVKSPLVCAINNAFSRYSISDNDLFRFNKKMFARRRILLKKNRHKRAGHGAKNKLKPISILTGKSERFRRKLIERWACEIADFFIKNKVGTVQMENLESMKRREDSYFNTRLRGFWPYAEMQNKIEFKLKQYGIEIRKVAPNNTSKTCSKCGHLNNYFNFEYRKRNKFPHFKCEKCNFKENADYNAALNISNPKLKSTKEEP

SEQ ID NO: 789 - protein, 726 aa, synthetic construct
SEVEFSHEYWMRHALMLAKRARDEREVPVGAVLVLNNRVIGEGWNRAIGLHDPTAHAEIMALRQGGLVMQNYRLIDATLYVTFEPCVMCAGAMVHSRIGRVVFGVRNSKRGAAGSLMNVLDYPGMDHRVEITEGILADECAALLCDFYRMPRQVFNAQKKAQSSINSGGSSGGSSSSETPGTSESATSESSGGSSGGSARNTITKTLQLRIVRPYNSAEVEKIVADEKNRREKIALEKNKGKVREACNKHLKVASYCTTQVERNACPFCKARKLDDKFYQKLRGQFPDAVFWQELGEILRQLQKQAAEIYNQSLIELYYEIFIKGRGFANASSVEHYLSDVCYTRAAELFKNAAIASGLRGKVKSNFRLKELKNMKSGLPTTKSDNFPIPLVRQKGGQYTGFEISSHNDDFIIKIPFGRWQVKKEIDKYRPWEKFDFEQVRKSPKPISLLLSTQRRKRNKGWSKDEGTEAEIRKVMNGDYQTSYIEVKRGSKTGEKSAWMLNLSIDVPKIDKGVDPSIIGGIDVGVKSPLVCAINNALSRYSISDNDLFRFNKKMFARRRILLKKNRHKRAGHGAKNKLKPISILTGKSERFRKKLIERWACEIADFFIKNKVGTVQMENLESMKRKEDSYFNIRLRGFWPYAEMQNKIEFKLKQYGIEIRKVAPNNTSKTCSKCGHLNNYFNFEYRKKNKFPHFKCEKCNFKENADYNAALNISNPKLKSTKEEP

SEQ ID NO: 790 - protein, 726 aa, synthetic construct
SEVEFSHEYWMRHALTLAKRARDEREVPVGAILVLNNRVIGEGWNRAIGLHDPTAHAEIMALRQGGLVMQNYRLIDATLYVTFEPCVMCAGAMIHSRIGRVVFGVRNSKHGAAGSLVNVLNYPGMNHRVEITEGILADECAALLCDFYRMPRQVFNARKKAQSSINPSGSSGGSSSSETPGTSGSATPEGSGGSSGGSAKNTITKTLKLRIVRPYNSAEVEKIVADEKNNREKIALEKNKDKVKEACSKHLKVASYCTTQVERNACLFCKARKLDDKFYQKLRGQFPDAVFWQELGEIFRQLQRQAAEIYNQSLIELYYEIFIKGKGFANASSVEHYLSDVCYTRAAELFKNAAIASGLRGKVKSNFRLKELKNMKSGLPTTKSDNFPIPLVKQKGGQYTGFEISSHNDDFIIKIPFGRWQVKKEIDRYRPWEKFDFEQVRKSPKPISLLLSTQRRKRNKGWSKDEGTEAEIRKVMNGDYQTSYIEVKRGSKIGEKSAWMLNLSIDVPKIDKGVDPSIVGGIDVGVKSPLVCAINNALSRYSISDNDLFHFNKKMFARRRILLKKNRHRRAGHGAKNKLRPITILTEKSKRFRRKLIERWACEIADFFIKNKVGTVQMENLESMKRKEDSYFNIRLRGFWPYAEMQNKIEFKLKQYGIEIRKVAPNNTSKTCSKCGHLNNYFNFEYRKKNKFPHFKCEKCNFKENADYNAALNISNPKLKSTKGEP

SEQ ID NO: 791 - protein, 726 aa, synthetic construct
SEVEFSHEYWMRHALTLAKRARDEREVPVGAVLVLNNRVIGEGWNRTTGLHDPTAHAEIMALRQGGLVMQNHRLVDATLYVTFEPCVMCAGAMIHSRIGRVVFGVRNSKRGAAGSLTNVLNYPGMNHRVEITEGILVDECAALLCDFYRMPRQVLNAQKKAQSSISPGGSSGGSSGSETPGASGSVTPKSSGGSSAGSTKDTITKTLKLRIVRPYNSAEVEKIVADEKNNREKIALEKNKDKVREACSKHLKVASYCTTQVERNACPFCKARKLDDKFYQKLRGQFPDAVFWQELGEILRQLQKQAAEIYNQSLIELYYEIFIKGRGFANASSVEHYLSDVCYTRAAELFKNAAIASGLRGKVKSNFRLKELKNMRSGLPTTKSDNFPIPLVKQKGGQYTGFEISSHNDDFIIKIPFGRWQVKEEIDKYRPWEKFDFAQVRKSPKPISLLLSTQRRKRNRGWSKDEGTEAEIKRVMSGDYQTSYIEVKRGSKIGEKSAWMLNLSIDVPKIDKGVDPSIIGGIDVGVKSPLVCAINNAFSRYSISDNDLFHFNKKMFARRRILLKKSKHKRAGHGAKSKLKPITILTEKSGRFRKKLIERWACEIADFFIKNKVGTVQMENLESMKRKEDSYFNIRLRGFWPYAEMQNKIEFKLKQYGIKIRKVAPNNTSKTCSKCGHLNNYFSFEYRKKNKFPHFKCEKCNFKEDADYNAALNISNPKLKSTKEEP

SEQ ID NO: 792 - protein, 726 aa, synthetic construct
SEVEFSHEYWMRRALTLAKRARDEREVPVGAVLVLNNRVIGVGWNRAVGLHDPTAHAEIMALRQGGLVMQNYRLVEATLYVTFEPCIMCAGAMIHSRIGRVVFGVRNSKRGAAGSLMNVLNYPGMNHRVEITEGILADECAALLCDFYRMPRQVFNARKKAQSSINPSGSSGGSSGSVTPGTSESATPESSGGGFGGSAKNTITKTLQLRIVRPYNSAEVEKIVADEKNNREKIALEKNKDKVKEACSKHLKVASYCTTQVERNACLFCKARKLDDKFYQKLRGQFPDAVFWQELGEIFRQLQKQAAEIYNQSLIELYYEIFIKGKGIANASSVEHYLSDVCYTRAAELFKNAAIASGLRNKIKSNFRLKELRNMKSGLPTTKSDNFPIPLVRQKGGQYTGFEISNHNGDFIIKIPFGRWQVKKEISKHRPWEKFDFEQVRKSPKPISLLLSTQRRKRNKGWGKDEGTEAEIRKVMNGDYQTSYIEVKRGSKIGEKSAWMLNLSIDVPKVDKGVDPNIIGGIDVGVKSPLVCAINNALSRYSISDNDLFHFNKKMFARRRILLRKNRYKRAGHGARNKLKPITVLTEKSERFRKKLIERWACEIANFFIKNKVGTVQMEDLESMKRREDSYFNIRLRGFWPYAEMQSKIEFKLKQYGIKIRKVAPNNTSKTCSKCGHLNNYFSFEFRKKNKFPHFKCEKCNFKEDADYNAALNISNPKLKSTKEEP

SEQ ID NO: 793 - protein, 726 aa, synthetic construct
SEVEFSHEYWMRHALTLAKRARDEREVPVGAVLVLNNRVIGAGWNRAVGLHDPTAHAEIMALRQGGLVMQNYRLVEATLYVTFEPCIMCAGAMIHSRIGRVVFGVRNSKRGAAGSLMNVLNHPGMNHRVEITEGILADECAALLCDYYRMPRQVFNARKKAQPSINSGGSSDGGSGSETPGTSESATPESSGGSSGGSAKNTITKTLKLRIVRPYNSAEVEKIVADEKNNREKIALEKNKGKVKEACSEHLKVAAYCTTQVERNACPFCKARKLDDKFYRKLRGQFPDAVFWQEIGEIFRQLQKQAAEIYNQSLIELYYEILIKGKGITNASRVEHYLSDVCYTRAAELFKNAAIASGLRSKVRSNFRLKELKNMKSGLPTTKSDNFPIPLVKQKGGQYTGFEISSHNSDFIIKIPFGRWQEKEEIDKYRPWEKFDFEQVRKSPKPISLLLSTQRRKKNKGWSKDEGTEAEIRRVMNGDYQTSYIEVKRGSKIGEKSAWMLNLSIDVPKIDKGVDPNIIGGIDVGVKSPLVCAINNSSSRYSICDNDLFRFNKKMFARRRILLKKNRHKRAGHGAKNKLKPITILTGKSVRFRKKLIERWACEIADFFIKNKVGTVQMENLESMKRKEDSYFNIRLRGFWPYAEMQNKIEFKLKQYGIEVRKVTPNNTSKTCSRCGHLNNYFSFEYRKKNKFPHFKCEKCNFKEDADYNAALNISNPKLKSTREEP

SEQ ID NO: 794 - protein, 726 aa, synthetic construct
SEAESSHEYWMRRALTLAERARDEREVPVGAVLVLNNRVIGVGWNRAIGLHDPTAHAEIMALRQGGLVTQNYRLIDATLYVTFEPCIMCAGAMIHSRIGRVVFGVRNSKRGAAGSLMNVLNYPGMNHRVEITEGILADECAALLCDYYRMPRQVFNAQKKAQSSINSGGSSGGSSGSKTPGASGSVIPKSSGGSSAGSTKDTITKTLKLRIVRPYNSAEVEKVVADEKNNREKIAMEKNKDKVKEACSKHLKVASYCTTQVERNACLFCKARKLDDKFYQKLRGQFPDAVFWQELGGIFRQLQKQAAEIYNQSLIELYYEIFIKGKGITNASRVEHYLSDVCYTRAAELFKNAAIASGLRSKVRSNFRLKELKNMKSGLPTTKSDNFPIPLVKQKGGQYTGFEISSHNDDFIIKIPFGRWQAKKEIDKYRPWEKFDFEQVRKSPKPISLLLSTQRRKRNKGWSKDEGTEAEIKKVMNGDYQISYIEVKRGSKIGEKSAWMLNLSVDVPKIDKGVDPSIIGGIDVGVKSPLVCAINNSFSRYSICDNDLFRFNKKMFARRRILLKKNRHKRAGHGAKNKLKPITILTKKSERFRKKLIERWVCEVADFFIKNKVGTVQMENLESMKRKEDSYFNIRLRGFWPYAEMQNRIELKLKQYGIEIRRVAPNNTSRTCSKCGHLNNYFNFEYRKKNKFPHFKCEKCNFREDADYNAALNISNPKLKSTKEEP

SEQ ID NO: 795 - protein, 726 aa, synthetic construct
SEVEFSHEYWMRHALTLAKRARDEGEVPVGAVLVLNNRVIGEGWNRAIGLHDPTAHAEIMALRQGGLVMQNYRLVDATLYVTFEPCVLCAGAMVHSRISRVVFGVRNSKRGAAGSLMNVLNNPGMNHRVEITEGILADECAALLCDFYRMPRQVFNAQKKARSNINSGSSSGGSSGSKTPGTSESATPEGSGGSSDGSAKNTITKTLKLRIVRPYNSAEVEKIVADEKNNREKIALEKNKDKVKEACSKHLKVASYCTTQVERNACLFCKARKLDDKFYQKLRGQFPDAVFWQELGEIFRQLQKQAAVVYNQSLIELYYEVFIKGKGFANASSVEHYLSDVCYTRAAELFKNAAIASGLRGKVKSNFRLKELKNMKSGLPTTKSDNFPIPLVKQKGGQYTGFEISSHNDDFIIKIPFGRWQVKKEIDKYRPWEKFDFEQVRKSPKPISLLLSTQRRKRNKGWSKDEGTEAEIRKVMNGDYQTSYIEVKRGSKIGEKSAWMLNLSIDVPKIDKGVDPSIIGGIDVGVKSPLVCAINNAFSRYSISDNDLFHFNKKMFARRRILLKKNRHKRAGHGTKNKLKPITILTEKSKRFRKKLIERWACEIADFFIKNKVGTVQMENLESMKRKEDSYFNIRLRGLWPYAEMQNKIEFKLKQYGIEIRKVAPNNTSKTCSKCGHLNNYFSFEYRKKNKFPHFKCEKCNFKEDADYNAALNISNPKLKSTKEEP

SEQ ID NO: 796 - protein, 726 aa, synthetic construct
SEVEFSHEYWMRHALTLAKRARDEREVPVGAVLVLNNRAIGEGWNRAIGLHDPTAHAEIMALRQGGLVMQNYRLTDATLYVTFEPCVMCAGAMIHSRIGRVVFGVRNSKRGAAGSLMNVLNYPGMNHCVEITEGILVDECAALLCDFYRMPRQVLNAQKKAQSSISSGGSSGGSSGSETPGASGSVIPKSSGGSSAGSTKDTITKTLKLRIVRPYNSAEVEKIVADEKNSREKIALEKNKDKVKEACSEHLKVAAYCTTQVERNACLFCKARKLDDKFYQKLRGQFPDAVFWQEIGEIFRQLQKQAAEIYNQSLIELYYEIFIKGRGFANASSVEHYLSDVCYTRAAELFKNAAIASGLRGKVKSNFRLKELKNMKSGLPTTKSDNFPIPLVKQKGGQYAGFEISSHNDDFIIKIPFGRWQVKKEIDKYRPWEKFDFEQVRKSPKPISLLLSTRRRKRNKGWSKDEGTEAEIRKVMNGDYQTSYIEVKRGSKIGEKSAWMLNLSIDVPKIDKGVDPSIIGGIDVGVKSPLVCAINNAFGRYSISDNDLFHFNKKMFARRRILLKRNRHKRAGHGAKNKLKPITILTEKSKRFRRKLIERWACEIADFFIKNKVGTVQMENLEGMKRKEDSYFNIRLRGFWPYAEMQNKIEFKLKQYGIEIRKVAPNNTSKTCSKCGHLNNYFNFEYRKKNKFPHFKCEKCNFKENADYNAALNISNPKLKSTKEEP

SEQ ID NO: 797 - protein, 726 aa, synthetic construct
SEVEFSHEYWMRHALTLAKRARDEREVPVGAILVLNNRVIGVGWNRAIGLHDPTAHAEIMALRQGGLVMQNYRLIDATLYVTFEPCVMCAGAMIHSRIGRVVFGVRNSKRGAAGSLMNVLNYPGMNHSVEITEGILVDECAALLCDFYRMPRQVLNAQKKAQSSISSGGSSGGSSGSETPGASGSVIPKSSGGSSAGSTKDTITKTLKLRIVRPYNSAEVEKVVADEKNNREKIAMEKNKDKVKEACSKHLKVASYCTTQVERNACLFCKARKLDDKFYQKLRGQFPDAVFWQELGGIFRQLQKQAAEIYNQSLIELYYEIFIKGKGITNASRVEHYLSDVCYTRAAELFKNAAIASGLRSKVRSNFRLKELKNMKSGLPTTKSDNFPIPLVKQKGGQYTGFEISSHNSDFIIKIPFGRWQVKEEIDKYRPWEKFDFEQVRKSPKPISLLLSTQRRQKNKGWSKDEGTEAEIRRVMNGDYQTSYIEVKRGGKIGEKSTWMLNLSIDVPKIDKGVDPSIVGGIDVGVKSPLVCAINNSFSRYSICDNDLFRFNKKMFARRRILLKKNRHKRAGHGAKNKLKPITILTKKSERFRKKLIERWVCEIADFFVKNKVGTVQMENLESMKRKEDSYFNIRLRGFWPYAEMQNKIEFKLKQYGIEIRKVAPNNTSKTCSKCGHLNNYFNFEYRRKNKFPHFKCEKCNFKENADYNAALNISNPKLKSTKEEP

SEQ ID NO: 798 - protein, 726 aa, synthetic construct
SEVEFSHEYWMRHALTLAKRARDEREVPVGAVLVLNNRVIGEGWNRAIGMHDPTAHAEIMALRQGGLVMQNYRLVDATLYVTFEPCVLCAGAMVHSRIGRVVFGVRNSKRGAAGSLMNVLNYPGMNHRVEITEGILADECAALLCDFYRMPRQVFNARKKAQSSINSGGSSGGSSGSETPGASESVTPKSSGGSSAGSTKNTITKTLKLRIVRPYNSAEVEKIVADEKNSREKIALERNKDKVKEACSEHLKVAAYCTTQVERNACLFCKARKLDDRFYQKLRGQFPDAVFWQELGEIFRQLQKQTAEIYNQSLIELYYEIFIKGKGITNASRVEHYLSDVCYTRAAELFKNAAIASGLRSKVRSNFRLKELKNMKSGLPTTKSDNFPIPLVKQKGGQYTGFEISSHNSDFIIKIPFGRWQVKEEIDKYRPWEKFDFEQVRKSPKPISLLLSTRRRKRNKGWSKDEGTEAEIRKVMNGDYQTSYIEVKRGSKIGEKSAWMLNLSIDVPKVDKGVDPSIIGGIDVGVKSPLVCAINNAFSRYSISDNELFHFNKKMFARRRILLKKNRHKRAGHGAKNKLKPISVLTEKSGRFRKKLIERWACEIADFFIKNKVGTVQMENLGSMKRKEDSYFNIRLRGFWPYAEMQNKIEFKLKQYGIEIRKVAPDNTSKTCSKCGHLNNYFNFEYRKKNKFPHFKCEKCNFKEDADYNAALNISNPKLKSTKEEP

SEQ ID NO: 799 - protein, 726 aa, synthetic construct
SEVEFSHEYWMRRALTLAKRARDEREVPVGAVLVLNNRVIGVGWNRAVGLHDPTAHAEIMALRQGGLVMQNYRLTDATLYVTFEPCVMCAGAMIHSRIGRVVFGVRNSKRGAAGSLMNVLNYPGMNHCVEITEGILVDECAALLCDFYRMPRQVLNAQKKAQSSISSGSSSGGSSGSETPDTSESATPESSGGSSGGSAKNTITKTLKLRIVRPYNSAEVEKIVADEKNNREKIALEKNKAKVKEACSEHLKMASYCTTQVERNACLFCKARKLDDKFYQKLRGQFPDAVFWQELGGIFRQLQKQAAEIYNQSLIELYYEIFIKGKGITNASRVEHYLSDVCYTRAAELFKNAAIASGLRSKVRSNFRLKELKNMKSGLPTTKSDNFPIPLVKQKGGQYTGFEISSHNSDLIIKIPFGRWQVKEEIDKYRPWEKFDFEQVRKSPKPISLLLSTQRRKRNKGWSKDEGTEAEIRKVMNGDYQTSYIEVKRGSKIGEKSAWMLNLSIDVPKVDKGVDPSIIGGIDVGVKSPLVCAINNAFSRYSISDNDLFRFNKKVFARRRILLKKNRHKRAGHGTKNKLKPITILTEKSGRFRKKLIERWACEIANFFVKNKVGTVQMEDLESMKRKEDSYFNIRLRGFWPYAEMQNKIEFKLKQYGIKIRKVAPNNTSKTCSKCGHLNNYFNFEYRKKSKFPHFKCEKCNFKEDADYNAALNISNPKLKSTKEEP

SEQ ID NO: 800 - protein, 726 aa, synthetic construct
SEVEFSHEYWMRHALTLAKRARDEREVPVGAVLVLNNRVIGEGWNRTTGLHDPTAHAEIMALRQGGLVMRNYRLTDATLYVTFEPCVMCAGAMIHSRIGRVVFGVRNSKRGAAGSLMNVLNYPGMNHCVEITEGILVDECAALLCDFYRMPRQVLNAQKKALSTINSGGSSGGSSGSETPGTSESPTPESSGGSPGGSAKNTITKTLKLRIVRPYNSAEVEKIVADEKNNREKIALEKNKDKVKEACSKHLKVAAYCTTQVERNACLFCKARKLDDGFYQKLRGQFPDAVFWQEIGEIFRQLQKQAAEIYNQSLIELYYEIFIKGKGFANASSVEHYLSDVCYTRAAELFKNAAIASGLRGKVKSNFRLKELKNMKSGLPTTKSDNFPIPLVKQKGGQYTGFEISSHNDDFIIKIPFGRWQVKKEIDKYRPWEKFDLEQVRKSPKPISLLLSTQRRKRNKGWSKDEGTEAEIRKVMNGDYQTSYIEVKRGSKIGEKSAWMLSLSIDVPKIDKGVDPSIIGGIDVGVKSPLVCAINNAFNRYSISDNNLFHFNKKMFARRRILLKKNRHKRAGHGAKNKLKPISILTEKSERFRKKLIERWACEIADFFIRNKVGTVQMENLEGMKRKEDSYFNIRLRGFWPYAEMQNKIEFKLKQYGIEVRKVAPNNTSKTCSKCGHLNNYFNFEYRKKNKFPHFKCEKCNFKENADYNAALNISNPKLKSTKGEP

SEQ ID NO: 801 - protein, 726 aa, synthetic construct; identical to SEQ ID NO: 88

SEQ ID NO: 802 - protein, 726 aa, synthetic construct
SEVEFSHEYWMRHALTLAKRARDEREVPVGAVLVLNNRVIGEGWNRAIGLYDPTAHAEIMALRQGGLVMQNYRLTDATLYVTFEPCVMCAGAMIHSRIGRVVFGVRNSKRGAAGSLMNVLNYPGMNHCVEITEGILVDECAALLCDFYRMPRQVLNAQKKAQPSISSGGSSGGSSGSETPGASESVTPKSSGGGSAGSTKNTITKTLKLRIVRPYNSAEVEKIVADEKNSRERIALEKNKDKVKEACSKHLKVAAYCTTQVERSACLFCKARRLDDKFYQKLRGQFPDAVFWQELGGIFRQLQKQAAEIYNQSLIELYYEIFIKGKGITNASRVEHYLSDVCYTRAAELFKNAAIASGLRGKVKSNFRLKELKNMKSGLPTTKSDNFPIPLVKQKGGQYTGFEISSHDDDFIIKIPFGRWQAKKEIDKYRPWEKFDFEQVRKSPKPISLLLSTQRRKRNKGWSKDEGTEAEIRKVMNGDYQTSYIEVKRGSKIGEKSAWMLNLSIDVPKIDKGVDPSIIGGIDVGVKSPLVCAINNAFSRYSISDNDLFRFNKKMFARRRILLKKNRHKRAGHGAKNKLKPISILTGKSERFRKKLIERWACEIADFFTKNKVGTVQMENLESMKRKEDSYFNIRLRGFWPYAEMQNKIEFKLKQYGIEIRKVAPNNTSKTCSKCGHLNNYFNFEYRKKNKFPHFRCKKCNFKENADYNAALNISNPKLKSTKEEP

SEQ ID NO: 803 - protein, 726 aa, synthetic construct
SEVEFSHEYWMRHALTLAKRARDEREVPVGAVLVLNNRVIGVGWNRAIGLHDPTAHAEIMALRQGGLVMQNYRLTDATLYVTFEPCVMCAGAMVHSRIGRVVFGVRNSKRGAAGSLMNVLNYPGMSHCVEITEGILVDECAALLCDFYRMPRQVLNAQKKAQSSISSGGSSGGSGGGETPGASESVTPKSSGGSSGSSAKNTITKTLKLRIVRPYNSAEVEKIVADEKNNREKIALEKNKDKVKEACSKHLKVAAYCTTQVERNACLFCKARRLDDKFYQKLRGQFPDAVFWQEIGEIFRQLQKQAAEVYNQSLVELYYEILIKGKGIANASSVEHYLSDVCYTRAAELFKNAAIASGLRGKVKSNFRLKELKNMKSGLPTTKSDNFPVPLVKQKGGQYTGFEISSHNDDFIIKIPFGRWQVKKEIDKYRPWEKFDFEQVRKSPKPISLLLSTQRRKRNKGWSKDEGTEAEIRKVMNGDYQTSYIEVKRGSKTGEKSAWMLNLSIDVPKIDKGVDPSIIGGIDVGVKSPLVCAINNAFSRYSISDNDLFRFNKKMFARRRILLRKNRHKRAGHGAKNKLKPISILTGKSERFRKKLIERWACEIADFFIKNKVGTVQMENLESMKRKEDSYFNIRLRGFWPYAEMQNKIEFKLKQYGIEIRKVAPNNTSKTCSKCGHLNNYFNFEYRKKNKFPHFKCEKCNFKENADYNAALNISNPKLKSTKKEP

SEQ ID NO: 804 - protein, 726 aa, synthetic construct
SEVEFSHEYWMRHALTLAKRARDEREVPVGAILVLNNRVIGEGWNRTTGLHDPTAHAEIMALRQGGLVMQSHRLVDATLYVTFEPCVMCAGAMIHSRIGRVVFGVRNSKRGAAGSLTNVLNYPGMNHCVEITEGILVDECAALLCDFYRMPRQVLNAQKKAQSSISSGGSSGGSSGSETPGASESVTPESSGGSPGGSAKNTITKTLKLRIVRPYNSTEVEKIVADEKNNREKIALEKNKDKVKEACSKHLKVAAYCTTQVERNACLFCKARRLDDKFYQKLRGQFPDAVFWQEIGEIFRQLQKQAAEIYNQSLIELYYEIFIKGKGFANASSVEHYLSDVCYTRAAELFKNAAIASGLRGKVKSNFRLKELKNMKSGLPTTKSDNFPIPLVKQKGGQYTGFEISSHNDDFIIKIPFGRWQVRKEIDKYRPWEKFNFEQVRKSPKPISLLLSTQRRKRNKGWSKDEGTEAEIRKVMNGDYQTSYIEVKRGSKIGEKSAWMLSLSIDVPKIDKGVDPSIIGGIDVGVKSPLVCAINNASSRYSISDNDLFRFNKKMFARRRILLKKSKHKRAGHGAKNKLKPITILTEKSRRFRKKLIERWACEIADFFIKNKVGTVLMENLESMKRKEDSYFNIRLRGFWPYAEMQNKIEFKLKQYGIVVRKVAPNNTSKTCSKCGHLNNYFNFEYRRKNKFPHFKCEKCNFKENADYNAALNICNPKLKSTKEEP

SEQ ID NO: 805 - protein, 726 aa, synthetic construct
SEVEFSHEYWMRHALALAKRARDAREVPVGAILVLNNRVIGEGWNRAIGQHDPTAHAEIMALRQGGLVMQNYRLIDATLYVTFEPCVMCAGAMIHSRIGRVVFGVRNSKHGAAGSLMNVLNYPGMNHRVEITEGILADECAALLCDFYRMPRQVFNGRKKAQSSINSGGSSGGSSGSEAPGTSESATPESSGGSSGGSAKNTITKTLQLRIVRPYNSAEVEKFVADEKNNREKIALEKNKDKVKEACSQHLKMASYCTTQVERNACLFCKARKLDDKFYQKLRGQFPDAVFWQELGEILRQLQKQAAEIYNQSLIELYYEIFIKGKGFANASSVEHYLSDVCYTRAAELFKNAAIASGLRGKVKSNFRLKELKNMKSGLPTTKSDNFPIPLVKQKGGQYTGFEISNHNSDFIIKIPFGRWQAKKEIDKYRPWEKFDFEQVRKSPKPISLLLSTQRRKRNKGWSKDEGTEAEIRKMMNGDYQTSYIEVKRGSKIGEKSAWMLNLSIDVPKIDKGVDPSIIGGIDVGVKSPLVCAINNAFSRHSISDNDLFHFNKKMFARRRILLKKNRHKRAGHGAKNKLKPISILTEKSKRFRKKLIERWACEIADFFIKNKVGTVQMENLESMKRKEDSYFNIRLRGFWPYAEMQNKIEFKLKQYGIEIRKVAPNNTSKTCSKCGHLNSYFDFEYRKKNKFPHFKCEKCNFKENADYNAALNISNPKLKSTKEEP

SEQ ID NO: 806 - protein, 726 aa, synthetic construct
SEVEFSHEYWMRHALTLAKRARDEREVPVGAILVLNNRVIGEGWNRAIGLHDPTAHAEIMALRQGGLVLQNYRLVDATLYVTFEPCVLCAGAMVHSRIGRVVFGARNSKRGAAGSLMNILNYPGMNHRVEITEGILADECAALLCDFYRMPRQVFSAQKKAQSSINSGGSSGGSSGSETPSTSESATPESSGGSSGGSAKNTITKTLQLRIVRPYNSAEVEKIVTDEKNNREKIALEKNKDKVKEACSKHLKMASYCTTQVERNACLFCKARKLDDKFYQKLRGQFPDAVFWQELGEIFRQLQKQAAEIYNQSLIELYYEIFIKGKGFANASSVEHYLSDVCYTRAAELFKNAAIASGLRGKVKSNFRLKELKNMKSGLPTTKSDNFPIPLVKQKGGQYTGFEISSHNDDFVIKIPFGRWLVKKEINKYRPWEKFDFEQVRKSPKPISLLLSTQRRKRNKGWSKDEGTEAEIRKVMNGDYQTSYIEVKRGSKTGEKNAWMLSLSIDVPKIDKGVDPSVIGGIDVGVKSPLVCAINNAFSRYSISDNDLFHFNKKMFARRRILLKKNRHKRAGHGAKNKLKPISILTERSKRFRKKLIERWACEIADFFIKNKVGTVQMENLESMKRKEDSYFNIRLRGFWPYAEMQNKIEFKLKQYGIEIRKVAPNNTSKTCSKCGHLNNYFNFEYRKMNKFPHFKCERCNFKENADYNAALNISNPKLKSTKEEP

SEQ ID NO: 807 - protein, 726 aa, synthetic construct
SEVEFSHEYWMRHALTLAKRARDEREVPVGAILVLNNRVIGEGWNRAIGLHDPTAHAEIMALRQGGLVMQNYRLTDATLYVTFEPCVMCAGAMIHSRIGRVVFGVRNSKRGAAGSLMNVLNYPGMNHCVEITEGILVDECAALLCDFYRMPRQVLNAQKKAQSSISSGGSSGGSSGSETPGASGSVTPKSSGGSSAGSTKDTITKTLKLRIVRPYNSAEVEKIVADEKNSREKIALEKNKDKVKEACSKHLKVAAYCTTQVERNACLFCKARRLDDKFYQKLRGQFPDAVFWQEIGEIFRQLQKQAAEIYNQSLVELYYEIFIKGKGIANASSVEHYLSDVCYTRAAELFKNAAIASGLRNKIKSNFRLKELRNMKSGLPTTKSDNFPIPLVRQKGGQYTGFEISNHNGDFIIKIPFGRWQVKKEICKHRPWEKFDFEQVRKSPKPISLLLSTQRRKRNKGWGKDEGTEAEIRKVMNGDYQTSYIEVKRGSKIGEKSAWMLNLSIDVPKIDKGVDPSIIGGIDVGVKSPLVCAINNALSRYSISDNDLFHFNKKMFARRRILLRKNRHKRAGHGAKNKLKPITILTEKSGRFRKKLIERWACEIADFFIKNKVGTVQMENLESMKRREDSYFNIRLRGFWPYAEMQNKIEFKLKQYGIEIRKVAPNNTSKTCSKCGHLNDYFNFEYRKKNKFPLFKCEKCNFKEDADYNAALNISNPKLKSTKEEP

SEQ ID NO: 808 - protein, 726 aa, synthetic construct
SEVEFSHEYWMRHALTLAKRARDEREVPVGAILVLNNRVIGEGWNRAIGLHDPTAHAEIMALRQGGLVMQNYRLIDATLYVTFEPCVMCAGAMIHSRIGRVVFGVRNSKHGAAGSLVNVLNYPGMNHRVEITEGILADECAALLCDFYRMPRQVFNARKKAQSSINPSGSSGGSSGSVTPCANESATPKSSGGSSAGSTKNTITKTLKLRIVRPYNSAEVERIVADEKNNRERIALEKNKDKVKEACSKHLKVAAYCTTQVERNACLFCKARKLDDKFYQKLRGQFPDAVFWQETGEIFRQLQRQAAEIYNQSLIELYYEIFIKGKGFANASSVEHYLSDVCYTRAAELFKNAAIASGLRGKVKSNFRLKELKNMKSGLPTTKSDNFPIPLVKQKGGQYTGFEISSHNDDFIIKIPFGRWQVKKEIDKYRPWEKFDFEQVRKSPKPISLLLSTQRRKRNKGWSRDEGTEAEIRKVMNGDYQTSYIEVKRGSKIGEKSAWMLSLSIDVPKIDKGVDPSIIGGIDVGVKSPLVCAINNAFCRYSISDNDLFHFNKKMFARRRILLKKSRHKRAGHGARNKLKPISILTEKSKRFRKKLIERWACEIADFFIKNKVGTVQMENLESMKRKEDSYFNIRLRGFWPYAEMQNKIEFKLKQYGIKVRKVAPNNTSKTCSKCGHLNNYFSFEYRKKNKFPHFKCEKCNFKENADYNAALNISNPKLKSTKEEP

SEQ ID NO: 809 - protein, 726 aa, synthetic construct
SEVEFSHEYWMRHALTLAKRARDEREVPVGAVLVLNNRVIGEGWNRAIGLHDPTAHAEIMALRQGGLVMQNYRLVDATLYVTFEPCVMCAGAMIHSRIGRVVFGVRNNKHGAAGSLMNVLNYPGMNHRVEITEGILADECAALLCDFYRMPRQVFNARKKAQSSINPGGPSGGSSGSKTPGTSESATPGSSGGSSSGSAKNTITKTLQLRIVRPYNSAEVEKIVADEKNNREKIALEKNKGKVKEACSKHLKVATYCTTQVERNACLFCKARKLDDKFYQKLRGQFPDAVFWQEVGEIFRQLQKQAAEIYNQSLIELYYEIFIKGKGIANASSVGHYLSDVCYTRAAELFKNAAIASGLRGKIKSNFRLKELKNMKSGLPTTKSDNFPIPLVKQKGGQYTGFEISNHDSDFIIKIPFGRWQVKKEIDKYRPWEKFDFEQVRKSPKPISLLLSTQRRKRNKGWSKDEGTEAEIKRVMNGDYQISYIEVKRGSKIGEKSAWMLNLSIDVPKIDKGVDPSIIGGIDVGVKSPLVCAINNAFSRYSISDNDLFHFNKKMFARRRILLKKNRHKRAGHGAKNKLKPLTILTGKSKRFRKKLIERWACEIADFFIKNKVGTVQMENLESMKRREDSYFNIRLRGLWPYAEMQNKIEFKLRQYGIEIRKVAPNNTSKTCSKCGHLNNYFNFEYRKKNKFPHFKCEKCNYKENADYNAALNISNPKLKSTKEEP

SEQ ID NO: 810 - protein, 726 aa, synthetic construct
SEVEFSHEYWMRHALTLAKRARDEREVPVGAVLVLNNRVIGEGWNRAVGLHDPTAHAEIMALRQGGLVMQNYRLTDATLYVTFEPCVMCAGAMIHSRIGRVVFGVRNSKRGAAGSLMNVLNYPGMNHCVEITEGILVDECAALLCDFYRMPRQVLNAQKKAQSSISSGGSSGGSSCSETPGASESVTPKSSGGSSAGSTRNTITKTLKLRIVRPYNSAEVEKIVADEKNSREKIALEKNKDKVKEACSEHLKVAAYCTTQVERNACLFCKARKLDDQFYQKLRGQSPDAVFWQELGEIFRQLQKQAAEIYNQSLIELYYEIFIKGKGFANASSVEHYLSDVCYTRAAELFKNAAIASGLRGKVKSNFRLKELKNMKSGLPTTKSDNFPIPLVKQKGGQYTGFEISSHNDDFIIKIPFGRWQAKKEIDKYRPWEKFDFEQVRKSPKPISLLLSTQRRKRNRGWSKDESTEAEIKKVMNGDYQTSYIEVKRGSKVGEKSAWMLNLSIDVPKIDKGVDPSIIGGIDVGVKSPLVCAINNTFSRYSISDNDLFHFNKKMFARRRILLKKSKHKRAGHGAKNKLKPITILTEKSGRFRKKLIERWASEIADFFIKNKVGTVQMENLESMKRKEDSYFNIRLRGFWPYAEMQNKIEFKLKQYGIEVRKVAPNNTSKTCSKCGHLNNYFNFEYRKKNKFPHFRCEKCNFKENADYNAALNISNPKLKSTKEEP

SEQ ID NO: 811 - protein, 726 aa, synthetic construct
SEVEFSHEYWMRRALTLAKRARDEREVPVGAVLVLNNRVIGVGWNRAVGLHDPTAHAEIMALRQGGLVMQNYRLIEATLYVTFEPCIMCAGAMIHSRIGRVVFGVRNSKRGAAGSLMNVLNYPGMNHCVEITEGILVDECAALLCDFYRMPRQVLNAQKKAQSSISPGGSSGGSSGSETPGASGSVTPKSSGGSSAGSTKDTITKTLKLRIVRPYNSAEVEKIVADEKNSREKIALEKYKDKVKEACSEHLKVAAYCTTQVERNACLFCKARKLDDKFYQKLRGQFPDAVFWQELGEILRQLQKQAAEIYNQSLIELYYEIFIKGKGYANASSVEHYLSDVCYTRAAELFKNAAIASGLRGKVKSNFRLKELKNMKSGLPTTKSDNFPIPLVKQKGGQYTGFEISSHDDDFIIKIPFGRWQVKKEIDKYRPWEKFDFEQVRKSPKPISLLLSTQRRKRNRGWSKDESTEAEIKKVMNGDYQTSYIEVKRGSKIGEKSAWMLSLSIDVPKIDKGVDPSIIGGIDVGVKSPLVCAINNAFSRYSISDNDLFHFNKKMFARRRILLKKNRHKRAGHGAKNKLKPISILTEKSKRFRKKLIERWACEIADFFIKNKVGTVQMENLESMKRKEDSYFNIRLRGFWPYAEMQNKIEFKLKQYGIKIRKVAPNNTSKTCSKCGHLNNYFSFEYRKKNKFPRFKCEKCNFKEDADYNAALNISNPKLKSTKEEP

SEQ ID NO: 812 - protein, 726 aa, synthetic construct
SEDEFSHEYWMRHALTLAKRARDEREVPVGAVLVLNNRVIGVGWNRAIGLHDPTAHAEIMALRQGGLVMQNYRLTDATLYVTFEPCVMCAGAMVHSRIGRVVFGVRNSKRGAAGSLMNVLNYPGMDHRVEITGGILADECAALLCDFYRMPRRVFNAQKKAQPSINSGGSSGGSSGSVTPGTSESATPESSGGSFGGSAKNTITKTLQLRIVRPYNSAEVEKIVADEKNNREKIALEKNKDKVKEACSKHLKVAAYCTTQVERNACLFCKARKLDDKFYQKLRGQYPDAVFWQEISEIFRQLQKQAAVIYNQGLIELYYEIFIKGKGIANASRVEHYLSNVCYTRAAELFKNAAIASGLRNKIKSNFRLKELRNMKSGLPTTKSDNFPIPLVRQKGGQYTGFEISNHDGDFIIKIPFGRWRVKKEINKHRPWEKFDFEQVRKSPKPISLLLSTQRRKRNKGWSKDEGTEAEIRKVMNGDYQTSYIEVKRGSKIGEKSAWMLNLSIDVPKIDKGVDPGIIGGIDVGVKSPLVCAINNAFSRYSISDNDLFHFNKKMFARRRILLKKNRHKRAGHGAKNKLKPISILTEKSRRFRKKLIERWACEIADFFIKNKVGTVQMENLESMKRKEDSYFNIRLRGFWPYAEMQNKIEFKLKQYGIEIRKVAPNNTSKTCSKCGHLNNYFNFEYRRMNKFPHFKCEKCNFKENADYNAALNISNPKLKSTKEEP

SEQ ID NO: 813 - protein, 726 aa, synthetic construct
SEVEFSHEYWMRHALTLAKRARDEREVPVGAVLVLNNRVIGVGWNRAIGLHDPTAHAEIMALRQGGLVMQNYRLIDATLYVTFEPCVMCAGAMIHSRIGRVVFGVRNSKHGAAGSLVNVLNYPGMNHRVEITEGILADECAALLCDFYRMPRQVFNARKKAQSSINSGGSSGGSSGSETPGTSESATPESSGGSSGGSAKNTITKTLKLRIVRPYNSAEVERILADEKDNREKIALERNKDKVKEACSKHLKVAAYCTTQVERNACLFCRARKLDDKFYQKLRGQFPDAVFWQEIGEIFRQLQKQAAEIYNQSLIELYYEIFIKGKGFANASSVEHYLSDVCYTRAAELFKNAAIASGLRGKVKSNFRLKELKNMKSGLPTTKSDNFPIPLVRQKGGQYTGFEISSHNDDFIIKIPFGRWQVKKEIDKYRPWEKFDFEQVRKSPKPISLLLSTQRRKRNKGWSKDEGTEAEIRKVMNGDYQTSYIEVKRGSKIGEKSAWMLNLSIDVPKIDKGVDPSIIGGIDVGVKSPLVCAINNAFSRYSISDNDLFHFNKKMFARRRILLKKNRRRRAGHGAKNKLKPITILTEKSVRFRKKLIERWACEIADFFIKNKVGTVQMENLESMKRKEDSYFNIRLRGFWPYAEMQNKIEFKLKQYGIKIRKVAPNNTSKTCSKCGHLNNYFNFEYRKKNKFPHFKCEKCNFKEDADYNAALNISNPKLKSTKGEP

SEQ ID NO: 814 - protein, 726 aa, synthetic construct
SEVEFSHEYWMRHALTLARRARDEHEVPVGAILVLNNRVIGEGWNRAIGLHDPTAHAEIMALRQGGLVMQNHRLVDATLYVTFEPCVMCAGAMIHSRIGRVVFGVRNSKRGAAGSLTNVLNYPGMNHRVEITEGILVDECAALLCDFYRMPRQVFNARKKAQSSINPGGSFGGSSGSETPGTSESATLESSGGSSGGSAKNTITKTLKLRIVRPYNSAEVEKIVADEKNSREKIALERNKDKVKEACSEHLKVAAYCTTQVERNACLFCKARKLDDRFYQKLRGQFPDAVFWQELGGIFRQLQKQAAEIYNQSLIELYYEIFIKGKGITNASRVEHYLSDVCYTRAAELFKNAAIASGLRSKVRSNFRLKELKNMKSGLPTTKSDNFPIPLVKQKGGQYTGFEISSHDDDFIIKIPFGRWQAKKEIDKYRPWEKFDFEQVRRSPKPISLLLSTQRRKRNKGWSKDEGTEAEIRKVMNGDYQTSYIEVKRGSKIGEKSAWMLNLSIDVPKIDKGVDPSIIGGIDVGVKSPLVCAINNALSRYSISDNDLFHFNKKMFARRRILLRKNRHKRAGHGAKNKLKPITILTERSGRFRKKLIERWACEIADFFIKNKVGTVQMENLESMKRKEDSYFNIRLRGFWPYAEMQNKIEFKLKQYGIEIRKVAPNNTSKTCSKCGHLNNYFNFEYRKKNKFPHFKCEKCNFKENADYNAALNISNPKLKSTKEEP

SEQ ID NO: 815 - protein, 726 aa, synthetic construct
SEVEFSHEYWMRHALTLAKRARDEREVPVGAILVLNNRVIGVGWNRAIGLHDPTAHAEIMALRQGGLVMQNYRLIDATLYVTFEPCVMCAGAMIHSRIGRVVFGVRNSKHGAAGSLVNVLNYPGMNHRVEITEGILADECAALLCDFYRMPRQVFNARKKAQSSINSGGSSGGSSGSETPGASESVTPKSSGGSTAGSTKNTITKTLKLRIVRPYNSAEVEKIVADEKNNREKTALEKNKDKVKEACSKHLKVAAYCTTQVERSACLFCKARKLDDKFYQKLRGQFPDAVFWQEVGEIFRQLQKQAAEIYNQSLIELYYEIFIKGKGFANASSVEHYLSDVCYTRAAELFKNAAIASGLRGKVKSNFRLKELKNMKSGLPTTKSDNFPIPLVKQKGGQYTGFEISSHNDDFIIKIPFGRWQVKKEIDKYRPWEKFDFEQVRKSPKPISLLLSTQRRKRNKGWSKDEGTEAEIRKVMNGDYQTSYIEVKRGSKIGEKSAWMLSLSIDVPKIDKGVDPSTIGGIDVGVKSPLVCAINNAFCRYSISDNDLFHFNKKMFARRRILLGKNRHKRAGHGVKNKLKPITILTEKSGRFRKKLIERWACEIADFFVKNKVGTVQMENLESMKRKEDSYFNIRLRGFWPYAEMQNKIEFKLKQYGIKVRKVAPNNTSKTCSKCGHLNNYFSFEYRKKNKFPHFKCEKCNFKENADYNAALNISNPKLKSTKEEP

SEQ ID NO: 816 - protein, 726 aa, synthetic construct
SEVEFSHEYWMRHALTLAKRARDEREVPVGAVLVLNNRVIGEGWNRAIGLHDPTAHAEIMALRQGGLVMQNYRLIDATLYVTFEPCVMCAGAMVHSRIGRVVFGVRNSKRGAAGSLMNVLDYPGMGHRVEITEGILADECAALLCDFYRMPRQVFSAQKRAQSSINSGGSSGGSSVSDTPGTSESAAPESSGGGSSGSAKNTITKTLQLRIVRPYNSAEVEKIVADEKNNREKIALEKNKDKVREACSKHLKVASYCTTQVERNACPFCKARKLDDKFYQKLRGQFPDAVFWQELGEILRQLQKQAAEIYNQSLIELYYEIFIKGRGFANASSVEHYLSDVCYTRAAELFKNAAIASGLRGKVKGNFRLKELKNMKSGLPTTKSDNFPIPLVKQKGGQYTGFEISSHNDDFIIKIPFGRWQVKKEIDRYRPWEKFDFEQVRKSPKPISLLLSTQRRKKNRGWSKDEGTEAEIRKVMNGDYQTSYIEVKRGSKIGEKSAWMLNLSIDVPKIDKGVDPSIIGGIDVGVKSPLVCAINNAFSRYSISDNDLFRFNKKMFARRRILLRKNRHKRAGHGAKNKLKPISILTGKSERFRKKLIERWACEIADFFIKNKVGTVQMENLESMKRKEDSYFNIRLRGFWPYAEMQNKIEFKLKQYGIEIRKVAPNNTSKTCSKCGHLNNYFNFEYRKKNKFPHFKCEKCDFKENADYNAALNISNPKLKSTKEEP

SEQ ID NO: 817 - protein, 726 aa, synthetic construct
SEVEFSHEYWMRHALSLAKRARDEREVPVGAVLVLNNRIIGEGWNRAIGLHDPTAHAEIMALRQGGLVMQNNRLTDATLYVTFEPCVMCAGAMVHSRIGRVVFGVRNSKRGAAGSLMNVLNYPGVNHCVEITEGILVDECAALLCDFYRMPRHVLNAQKKAQSSISSGGSSGGCSGSEMPGASESVTPKSSGGSSAGSTKNTITKTLKLRIVRPYNSAEVEKIVADEKNSREKIALERNKDKVKEACSEHLKVAAYCTTQVERNACLFCKARKLDDRFYQKLRGQFPDAVFWQEIGEIFRQLQKQAAEIYNQSLIELYYEIFIKGKGFANASSVEHYLSDVCYTRAAELFKNAAIASGLRGKVKSNFRLKELKSMKSGLPTTKSDNFPIPLVKQKGGQYTGFEISSHNDDFIIKIPFGRWQAKKEIDKYRPWEKFDFEQVRKSPKPISLLLSTQRRKRNRGWSKDEGTEAEIRKVMNGDYQTSYIEVKRGSKIGEKSAWMLNLSIDVPKIDKGVDPSIIGGIDVGVKSPLVCAINNAFSRYSISDNDLFRFNKKMFARRRILLGKNRHKRAGHGVKNKLKPITILTEKSKRFRRKLIERWACEIADFFIKNKVGTVQMENLESMKRKEDSYFNIRLRGFWPYAEMQNKIEFKLKQYGIEIRKVAPNNTSKTCSKCGHLNNYFNFEYRRKNKFPHFKCEKCNFKEDADYNAALNISNPKLKSTKEEP

SEQ ID NO: 818 - protein, 726 aa, synthetic construct
SEVEFSHEYWMRHALTLAKRARDEREVPVGAVLVLNNRVIGEGWNRATGLHDPTAHAEIMALRQGGLVMQNYRLFDATLYVTFEPCVMCAGAMIHSRIGRVVFGVRNSKRGAAGSLMNVLNYPGMNHCVEITEGILVDECAALLCDFYRMPRQVFNARKKAQSSINPGGSFGGGSGSETPGTSESATLESSGGSSGGSAKNTITKTLKLRIVRPYNSAEVERIVADEKNSREKIALEKNKDKVKEACSRHLRVAAYCTTQVERNACLFCKARKLDDKFYQKLRGQFPDAVFWQEIGEIFRQLQKQAAEVYNQSLVELYYEILIKGKGIANASSVEHYLSDVCYTRAAELFKNAAIASGLRNKIKSNFRLKELRNMKSGLPTTKSDNFPIPLVRQKGGQYTGFEISNHDGDFIIKIPFGRWQVKKEINKHRPWEKFDFEQVRKSPKPISLLLSTQRRKRNKGWSKDEGTEAEIRKVMNGDYQTSYIEVKRGSKIGEKSAWMLNLSIDVPKIDKGVDPSIIGGIDVGVKSPLVCAINNALSRYSISDNDLFHFNKKMFARRRILLRKNRHKRAGHGVKNKLKPITILTEKSGRFRKKLIERWACEIADFFVKNKVGTVQMENLESMKRKEDSYFNIRLRGFWPYAEMQNKIEFKLKQYGIKVRKVAPNNTSKTCSKCGHLNNYFSFEYRKKNKFPHFKCEKCNFKENADYNAALNISNPKLKSTKEEP

SEQ ID NO: 819 - protein, 726 aa, synthetic construct
SEVEFSHEYWMRHALILAKRARDEREVPVGAVLVLNNRVIGVGWNRAIGLHDPTAHAEIMALRQGGLVMQNYRLIGATLYVTFEPCAMCAGAMIHSRIGRVVFGVRNSKRGAAGSLMNVLNYPGMNHRVEIMEGILTDECAALLCDFYRMPHQVLNAQRKAQSSINSGGSSGGSSGSETPGTSGSATPEGSGGSSAGSTKDTITKTLKLRIVRPYNSAEVEKIVADEKNSREKIALEKNKDKVKEACSEHLKVAAYCTTQVERNACLFCKARKLDDGFYQKLRGQFPDAVFWQEIGEIFRQLQKQAAEIYNQSLIELYYEIFIKGKGFANASSVEHYLSNVCYTRAAELFKNAAIASGLRGKVKGNFRLKELKNMKSGLPTTKSDNFPIPLVKQKGGQYTGFEISSHNDDFIIKIPFGRWQVKKEIDKYRPWEKFDFEQVRKSPKPISLLLSTQRRKRNKGWSKDEGTEAEIRKVMNGDYQTSYIEVKRGSKTGEKSAWMLNLSIDVPKIDKGVDPSIIGGIDVGVKSPLVCAINNAFSRYSISDNDLFRFNKKMFARRRVLLKKNRHKRAGHGAKNKLKPITILTEKSVRFRKKLIERWACEIADFFIKNKVGTVQMENLESMKGKEDSYFNIRLRGFWPYAEMQNKIEFKLKQYGIEIRKVAPNNTSKTCSKCGHLNNYFNFEYRKKNKFPHFKCEKCNFKENADYNAALNISNPKLKSTKEEP

SEQ ID NO: 820 - protein, 726 aa, synthetic construct
SEVEFSHEYWMRHALTLAKRARDEGEVPVGAVLVLNNRVIGEGWNRAIGLHDPTAHAEIMALRQGGLVIQNYRLVDATLYVTFEPCVLCAGAMVHSRIGRVVFGVRNSKRGAAGSLMNVLNYPGMNHRVEITEGILADECAALLCDFYRMPRQVLSAQKKAQSSVSSGGSSGGSSGSETPGASGSVTPKSSVGSSAGSTKNSITKTLKLRIVRPYNSAEVEKIVADEKNNREKIALEKNKGKVKEACSKHLKVATYCTTQVERNACLFCKARKLDDKFYQKLRGQFPDAVFWQEVGEIFRQLQKQAAEIYNQSLIELYYEIFIKGKGIANASSVGHYLSDVCYTRAAELFKNAAIASGLRGKIKSNFRLKELKNMKSGLPTTKSDNFPIPLVKQKGGQYTGFEISNHNGDFIIKIPFGRWQVKKEINKYRPWEKFDFEQVRKSPKPISLLLSTQRRKRNKGWSKDEGTEAEIKKVMNGDYQISYIEVKRGSKIGEKSAWTLNLSVDVPKIDKGVDPSIIGGIDVGVKSPLVCAINNALSRYSISDNDLFHFNKRVFARRRILLKKNRHRRAGHGAKNKLKPITILTEKSKRFRKKLIERWACEIADFFIKNKVGIVQMENLESMKRREDSYFNIRLRGFWPYAEMQNKIEFKLKQYGIEVRKVAPNNTSKTCSKCGHLNNYFNFEYRKKNKFPHFKCEKCNFKEDADYNAALNISNPKLKSTKEEP

SEQ ID NO: 821 - protein, 726 aa, synthetic construct
SEVEFSHEYWMRHALTLAKRARDEREVPVGAVLVLNNRVIGEGWNRTTGLHDPTAHAEIMALRQGGLVMRNYRLTDATLYVTFEPCVMCAGAMIHSRIGRVVFGVRNSKRGAAGSLMNVLNYPGMNHCVEITEGILVDECAALLCDFYRMPRQVLNAQKKAQSSINPGGSSGGSGGSETPGTSESATPESSGGSSGSSAKNTITKTLKLRIVRPYNSAEVEKIVADEKNNREKIALEKNKDKVKEACSEHLKVAAYCTTQVERNACLFCKARKLDDRFYQELRGQFPDAVFWQEIGEIFRQLQKQAAEIYNQSLIELYYEIFIKGKGFANASSVEHYLSDVCYTRAAELFKNAAIASGLRGKVKSNFRLKELKNMKSGLPTTKSDNFPIPLVRQKGGQYTGFEVSSHNDDFIIKIPFGRWQVKKEIDKYRPWEKFDFEQVRKSPRPISLLLSTQRRKRNKGWSKDEGTEAEIRKVMNGDYQTSYIEVTRGSKIGEKSAWMLNLSIDVPKIDKGVDPSIIGGIDVGVKTPLVCAINNAFSRYSISDNDLFHFNKKMFARRRILLKKSRHKRAGHGAKNKLKPITILTEKSKRFRKKLIERWACEIADFFIKNKVGTVQMENLESMKRKEDSYFNIRLRGFWPYAEMQNKIEFKLKQYGIEIRKVAPNNTSKTCSKCGHLNNYFNFEYRKKNKFPHFKCEKCNFKENADYNAALNISNPKLKSTKEEP

SEQ ID NO: 822 - protein, 726 aa, synthetic construct
SEVEFSHEYWMRHALTLAKRARDEREVPVGAILVLNNRVIGEGWNRAIGLHDPTAHAEIMALRQGGLVMQNYRLIDATLYVTFEPCVMCAGAMIHSRIGRVVFGVRNNKHGAAGSLVNVLNYPGMNHRVEITEGILADECAALLCDFYRMPRQVFNARKKAQSSISSGGTSGGCSGSEMPGASESVTPKCSGGSSAGSTKNTITKTLKLRIVRPYNSAEVEKIVADEKNNREKIALEKNKDKVKEACSKHLKVAAYCTTQVERNACPFCKARKLDDKFYQKLRGQFPDAVFWQELGEILRQLQKQAAEIYNQSLIELYYEIFIKGRGFANASSVEHYLSDVCYTRAAELFKNAAIASGLRGKVKSNFRLKELKNMRSGLPTTKSDNFPIPLVKQKGGQYAGFEISSHNDDFIIKIPFGRWQVKKEIDKYRPWEKFDFEQVRKSPKPISLLLSTRRRKRNKGWSKDEGTEAEIRKVMNGDYQTSYIEVKRGSKIGEKSAWMLNLSIDVPKIDKGVDPSIIGGIDVGVKSPLVCAINNAFSRYSISDNDLFHFNKKMFARRRILLKRNRHKRAGHGAKNKLKPISILTEKSKRFRKKLIERWACEIADFFIKNKVGTVQMENLESMKRREDSYFNIRLRGFWPYAEMQNKIEFKLKQYGIEIRKVAPNNTSKTCSKCGHLNNYFNFEYRKMNKFPHFKCEKCNFKENADYNAALNISNPKLKSTKEEP

SEQ ID NO: 823 - protein, 726 aa, synthetic construct
SEVEFSHEYWMRHALTLAKRARDGREVPVGAILVLNNRVIGEGWNRAIGLHDPTAHAEIMALRQGGLVMQNYRLIDATLYVTFEPCVMCAGAMIHSRIGRVVFGVRNSKHGAAGSLVNVLNYPGMNHRVEITEGILADECAALLCDFYRMPRQIFNARKKAQSSINPSGSSGGSSGSVTPGTSESATPESSGGGFGGSAKNTITKTLKLRIVRPYNSAEVEKIVADEKNNREKIALEKNKDKVKEACSKHLKVAAYCTTQVERNACLFCKARKLDDKFYQKLRGQFPDAVFWQELGEIFRQLQKQAAEIYNQSLIELYYEIFIKGKGFANASSVEHYLSDVCYTRAAELFKNAAIASGLRGKVKSNFRLRELKNMKSGLPTTKSDNFPISLVKQKGGQYTGFEISSHNDDFIIKIPFGRWQAKKEIDKFRPWEKFDFEQVRKSPKPISLLLSTQRRKRNKGWSKDEGTEAEIRKVMNGDYQTSYIEVKRGSKIGEKSAWMLNLSIDVPKIDKGVDPSIIGGIDVGVKSPLVCAINNAFSRYSISDNDLFHFNKKMFARRRILLKKNRHKRAGHGAKNKLKPISILTGKSKRFRKKLIERWACEIADFFIKNKVGTVQMENLESMRRKEDSYFNIRLRGFWPYAEMQNKIEFKLKQCGIVVRKVAPNNTSKTCSKCGHLNNYFNFEYRKKNKFPHFKCEKCNFKEDADYNAALNISNPKLKSTKGEP

SEQ ID NO: 824 - protein, 726 aa, synthetic construct
SEIEFSHEYWMRHALTLAKRARDEREVPVGAVLVLNNRVIGEGWNRAIGLHDPTAHAEIMALRQGGLVMQNYRLTDATLYVTFEPCVMCAGAMIHGRIGRVVFGARNSKRGAAGSLMNVLNYPGMNHCVKITEGILVDECAALLCDFYHMPRQVLNAQKKAQSSINPGGSSGGSSGSETPGTSESATPESSGGSSGSSAKNTITKTLKLRIVRPYNSAEVEKIVADEKNNREKIALEKNKDKVKEACSKHLKVAAYCTTQVERNACLFCKARRLDDKFYQKLRGQFPDAVFWQELGEIFRQLQKQAAEIYNQSLIELYYEIFIKGKGFANASSVEHYLSDVCYTRAAELFKNAAIASGLRGKVKSNFRLKELKNMKSGLPTTKSDNFPIPLVKQKGGQYTGFEISSHNDDFIIKIPFGRWQVKKEIDKYRPWEKFDFEQVRKSPKPISLLLSTRGRKRNKGWSKDEGTEAEIRKVMNGDYQTSYVEVKRGSKIGEKSAWMLSLSIDVPKINKGVDPSIIGGIDVGVKSPLVCAINNALSRYSISDNDLFHFNKKMFARRRILLKRNGHKRAGHGTKNKLKPITILTEKSVRFRKKLIERWACEIADFFIKNKVGTVQMENLESMKRKEDSYFNIRLRGFWPYAEMQNKIEFKLKQYGIEIRKVAPNNTSKTCSKCGHLNNYFNFEYRKKNKFPHFKCEKCNFKENADYNAALNISNPKLKSTKEGP

SEQ ID NO: 825 - protein, 726 aa, synthetic construct; identical to SEQ ID NO: 688

SEQ ID NO: 826 - protein, 726 aa, synthetic construct
SEVEFSHEYWMRHALTLAKRARDEREVPVGAILVLNNRVIGEGWNRAIGLHDPTAHAEIMALRQGGLVMQNYRLIDATLYVTFEPCVMCAGAMIHSRIGRVVFGVRNNKHGAAGSLVNVLNYPGMNHRVEITEGILADECAALLCDFYRMPRQVFNARKKVRSSINPGGSSGGSSGSETPSTSESATPESSGGSSGGSAKNTITKTLQLRIVRPYNSAEVEKIVTDEKNNREKIALEKNKDKVKEACSKHLKMASYCTTQVERNACLFCKARKLDDKFYQKLRGQFPDAVFWQELGGIFRQLQRQAAEIYNQSLIELYYEIFIKGKGITNASRVEHYLSDVCYTRAAELFKNAAIASGLRSKVRSNFRLKELKNMKSGLPTTKSDNFPIPLVKQKGGQYTGFEISSHNSDFIIKIPFGRWQVKEEIDKFRPWEKFDFEQVRKSPKPISLLLSTQRRKKNKGWSKDEGTEAEIRKVMNGDYQTSYIEVKRGSKIGEKSAWMLNLSIDVPKIDKGVDPSIIGGIDVGVKSPLVCAINNALSRYSISDNDLFHFNKKVFARRRILLKKNRHKRAGHGAKNKLKPITIMTEKSKRFRKKLIERWACEIADFFIKNKVGTVQMENLESMKRREDSYFNIRLRGFWPYAEMQNKIEFKLKQYGIVVGKVAPNNTSKTCSKCGHLNNYFNFEYRKKNKFPHFKCEKCNFRENADYNAALNISNPKLRSTKEEP

SEQ ID NO: 827 - protein, 726 aa, synthetic construct
SEVELSHEYWMRHALSLAKRARDEREVPVGAVLVLNNRVIGEGWNRAIGLHDPTAHAEIMALRQGGLVMQNHRLIDATLYVTFEPCVMCAGAMIHSRIGRVVFGVRNSKRGAAGSLMNVLNYPGMNHRVEITEGILTDECAALLCDFYRMPHQVLNAQKKAQSSINSGGSSGGSSGSETPGTGGSATPEGSGGSSGGFAKSTITKTLKLRIVRPYNSAEVEKIVADEKNNREKIALEKNKGKVKEACSKHLKVATYCTTQVGRNACLFCKARKLDDKFYQKLRGQFPDAVFWQEIGEIFRQLQKQAAEIYNQSLIELYYEIFIKGKGFANASSVEHYLSDVCYTRAAELFKNAAIASGLRGKVKSNFRLKELKNMKSGLPTTKSDNFPIPLVKQKGGQYTGFEISSHNDDFIIKIPFGRWQVKKEIDKYRPWEKFDFEQVRKSPKPISLLLSTQRRKRNKGWSKDEGTEAEIRKVMNGDYRTSYIEVKRGSKIGEKSAWMLNLSIDVPKIDKGVDPSIIGGIDVGVKSPLVCAINNAFSRYSISDNDLFRFNKRMFARRRILLKKSKHKRAGHGAKNKLKPITILTEKSGRFRKKLIERWACEIADFFIKNKVGTVQMENLESMKRKEDSYFNIRLRGFWPYAEMQNKIEFKLKQYGIEIRKVAPHNTSRTCSKCGHLNNYFNFEYRRKNKFPHFKCEKCNFKEDADYNAALNISNPKLKSTMEEP

SEQ ID NO: 828 - protein, 726 aa, synthetic construct
SEVEFSHEYWMRHALALAKRARDEREVPVGAVLVLNNRVIGEGWNRAIGLHDPTAHAEIMALRQGGLVMQNYRLVDATLYVTFEPCVLCAGAMVHSRIGRVVFGVRNSKRGAAGSLMNVLNYPGMNHRVEITEGILVDECAALLCDFYRMPRQVFNAQKKAQSTINSGGSSGGSSGSETPGTSESPTPESSGGSPGGSAKNTITKTLKLRIVRPYNSAEVEKIVADEKNNREKIALEKNKDKVKEACSEHLKVAAYCTTQVERNACLFCRARKLDDKFYQKLRGQFPDAVFWQEIGEIFRQLQKQAAEIYNQSLIELYYEIFIKGKGFANASSVEHYLSDVCYTRAAELFKNAAIASGLRGKVKSNLRLKELKNMKSGLPTTKSDNFPIPLVKQKGGQYTGFEISSHNDDFIIKIPFGRWQVKKEIDKYRPWEKFDFEQVRKSPKPISLLLSTQRRKRNKGWGKDEGTEAEIRKVMNGDYQTSYIEVKRGSKIGEKSAWMLSLSIDVPKIDKGVDPRIIGGIDVGVKSPLVCAVNNAFSRYSISDNDLFHFNKKMFARRRILLKKNRHKRAGHGAKSKLKPISILTEKSERFRKKLIERWACEIADFFIKNKVGTVQMENLESMKRKEDSYFNIRLRGFWPYAEMQNKIEFKLKQYGIKIRKVAPNNTSKTCSKCGHLNNYFSFEYRKKNKFPHFKCEKCNFKEDADYNAALNISNPKLKSTKEEP

SEQ ID NO: 829 - protein, 726 aa, synthetic construct
SEVEFSHEYWMRHALTLAKRARDEREVPVGAVLVLNNRVIGEGWNRAIGLHDPTAHAEIMALRQGGLVMQNYRLTDATLYVTFEPCVMCAGAMIHSRIGRVVFGVRNSKRGAAGSQMNVLNYPGMNHCVEITEGILVDECAALLCDFYRMPRQVLNAQKKAQSSISPGGSSGGSSGSETPGASGSVTPKSSGGSSAGSTKDTITKTLKLRIVRPYNSAEVEKIVADEKNNREKIALEKNKDKVKEACSKHLKVAAYCTTQVERNACLFCKARKLDDKFYQKLRGQFPDAVFWQEIGEIFRQLQRQAAEIYNQSLIELYYEIFIKGKGFANASSVEHHLSDVCYTRAAELFKNAAIASGLRGKVKSNFRLKELRNMKSGLPTTKSDNFPIPLVKQKGGQYTGFEISSHDDDFVIKIPFGRWQVKKEIDKYRPWEKFDFEQVRKSPKPISLLLSTQRRKRNKGWSKDEGTEAEIRKVMNGDYQTSYIEVKRGSKIGEKSAWMLNLSIDVPKIDKGVDPSIIGGIDVGVKSPLVCAINNAFSRYSISDNDLFHFNKKMFARRRILLKKNKHKRAGHGAKNKLKPISILTEKSGRFRKKLIERWACEIANFFIKNKVGTVQMENLEGMKRKEDSYFNIRLRGFWPYAEMQNKIEFKLKQYGIEIRKVAPNNTSKTCSKCGHLNNYFSFEYRKKNKFPHFKCEKCNFKENADYNAALNISNPKLKSTKEEP

SEQ ID NO: 830 - protein, 726 aa, synthetic construct
SEVEFSHEYWMRHALTLARRARDEREVPVGAVLVLNNRVIGEGWNRAIGLHDPTAHAEIMALRQGGLVMQNYRLTDATLYVTFEPCVMCAGAMIHSRIGRVVFGVRNSKRGAAGSLMNVLNYRGMNHCVEITEGILVDECAALLCDFYRMPRQVLNAQKKAQSSVSPGSSSGGSGGGGTPGASESVTPKNSGGSSAGSTKNTITKTLKLRIVRPYNSAEVEKIVADEKNSREKIALEKNKDKVKEACREHLKVAAYCTTQVERSACLFCKARKLDDRFYQKLRGQFPDAVFWQELGEIFRQLQKQAAEVYNQSLVELYYEILIKGKGIANASSVEHYLSDVCYTRAAELFKNAAIASGLRNKIKSNFRLKELRNMKSGLPTTKSDNFPIPLVRQKGGQYTGFEISNHDGDFIIKIPFGRWQVKKEINKHRPWEKFDFEQVRKSPKPISLLLSTQRRKRNKGWSKDEGTEAEIRKVMNGDYQTSYIEVKRGSKIGEKSAWMLNLSIDVPKIDRGVDPSITGGIDVGVKSPLVCAINNALSRYSISDNDLFHFNKKMFARRRILLRKNRHKRAGHGAKNKLKPISILTEKSKRFRKKLIERWACEIADFFIKNKVGTVQMENLESMKRKEDSYFNIRLRGFWPYAEMQNKIEFKLKQYGIEIRKVAPNNTSKTCSKCGHLNSYFDFEYRKKNKFPHFKCEKCNFKENADYNAALNISNPKLKSTKEEP

SEQ ID NO: 831 - protein, 726 aa, synthetic construct
SEVEFSHEYWMRHALTLAKRARDEREVPVGAVLVLNNRVIGEGWNRAIGLHDPTAHAEIMALRQGGLVMQNYRLTDATLYVTFEPCVMCAGAMIHSRIGRVVFGVRNSKRGAAGSLMNVLNYPGMNHCVEITEGILVDECAALLCDFYRMPRQVLNAQKKAQSSISSGGSSGGSSCSETPGDSESVTPKSSGGSSAGSTKNTITKTLKLRIVRPYNSAEVEKIVADEKNSREKIALEKNKDKVKEACSEHLKVAAYCTTQVERNACLFCKARKLDDRFYQELRGQFPDAVFWQETGEIFRQLQRQAAEIYNQSLIELYYEIFIKGKGFANASSVEHYLSDVCYTRAAELFKNAAIASGLRGKVKSNFRLKELKNMKSGLPTTKSDNFPIPLVKQKGGQYTGFEISSHNDDFIIKIPFGRWQVKKEIDKYRPWEKFDFEQVRKSPKPISLLLSTQRRKRNKGWSKDEGTEAEIRKVMNGDYQTSYIEVKRGSKIGEKSAWMLNLSIDVPKIDKGVDPSIIGGIDVGVKSPLVCAINNAFSRYSISDNDLFRFNKKVFARRRILLKKNRHKRAGHGTKNKLKPITILTEKSGRFRKKLIERWACEIANFFIKNKVGTVQMENLESMKRKEDSYFNIRLRGFWPYAEMQNKIEFKLKQYGIEIRKVAPNNTSKTCSKCGHLNNYFSFEYRKKNKFPHFKCEKCNFKEDADYNAALNISNPKLKSTKEEP

SEQ ID NO: 832 - protein, 726 aa, synthetic construct
SEVEFSHEYWMRHALTLAKRARDGREVPVGAVLVLNNRVIGEGWNRAIGLHDPTAHAEIMALRQGGLVMQNYRLIDATLYVTFEPCVMCAGAMVHSRIGRVVFGVRNSKRGAAGSLMNVLDYPGMGHRVEITEGILVDECAALLCDFYRMPRQVLNAQKKAQSSISFGGSSGGSSGSETPGASGSVTPKSSGGSSAGSTKDTITKTLKLRIVRPYNSAEVEKVVADEKNNREKIAMEKNKDKVKEACSKHLKVASYCTTQVERNACLFCKARKLDDKFYQKLRGQFPDAVFWQELGGIFRQLQKQAAEIYNQSLIELYYEIFIKGKGFANASSVEHYLSDVCYTRAAELFKNAAIASGLRGKVKSNFRLKELKNMKSGLPTTKSDNFPIPLVKQKGGQYTGFEISSHNDDFIIKIPFGRWQVKREIDKYRPWEKFDFEQVRKSPKPISLLLSTRRRKKNKGWSKDEGTEAEIRRVMNGDYQTSYIEVKRGSKIGEKSAWMLNLSIDVPKVDKGVDPSIIGGIDVGVKSPLVCAVNNSFSKYSICDNDLFRFNKKMFARRRILLKKNRHKRAGHGAKNKLKPITILTKKSERFRKKLIERWACEVADFFIKNKVGTVQMENLESMKRKEDSYFNIRLRGFWPYAEMQNKIEFKLKQYGIEIRRVAPNNTSRTCSKCGHLNNYFNFEYRKKNKFPHFKCEKCNFREDADYNAALNISNPKLKSTKEEP

SEQ ID NO: 833 - protein, 726 aa, synthetic construct
SEVEFSHEHWMRHALTLAKRARDEREVPVGAVLVLNNRVIGEGWNRAIGLHDPTAHAEIMALRQGGLVMQNYRLTDATLYVTFEPCVMCAGAMIHSRIGRVVFGVRNNKHGAAGSLVNVLNYPGMNHRVGITEGILADECAALLCDFYRMPRQVFNAQKKAQSSISSGGSSGGCSGSEMPGASESVTPKSSGGSPGGSAKNTITKTLKLRIVRPYNSAEVEKIVAEEKDNREKIALEKNKDKVREACSKHLKVAAYCTTQVERNACLFCKARKLDDKFYQKLRGQFPDAVFWQEIGEIFRQLQKQAAEIYNQSLIELYYEIFIKGKGFANASSVEHYLSDVCYTRAAELFKNAAIASGLRGKVKSNFRPKELKNMKSGLPTTKSDNFPIPLVKQKGGQYTGFEISSHNDDFIIKIPFGRWQVKKEIDKYRPWEKFDFEQVRKSPKPISLLLSTQRRKRNKGWSKDEGTEAEIRKVMNGDYQTSYIEVKRGSKIGEKSAWMLNLSIDVPKIDKGVDPSIIGGIDVGVKSPLVCAINNAFSRYSISDNDLFHFNKKMFARRRILLKKTRHKRAGHGAKNKLKPVSILTEKSERFRKKLIERWACEIADFFIKNKVGTVQMENLESMKRREDSYFNIRLRGFWPYAKMQNKIEFKLKQYGIEIRKVAPNNTSKTCSKCGHLNNYFNFEYRKKNKFPHFKCEKCNFKENADYNAALNISNPKLKSTKEGP

SEQ ID NO: 834 - protein, 726 aa, synthetic construct
SEVEFSHEYWMRHALTLAKRARDEREVPVGAILVLNNRVIGEGWNRAIGLHDPTAHAEIMALRQGGLVMQNYRLIEATLYVTFEPCIMCAGAMIHSRIGRVVFGVRNSKRGAAGSLMNVLNYPGMNHRVEITEGILADECAALLCDYYRMPRQVFNARKKAQSSINSGGSSGGSSGSETPGTSESPTPESSGGSPGGSAKNTITKTLKLRIVRPYNSAEVEKIVADEKNNREKIALEKNKDKVKEACSKHLKVAAYCTTQVERNACLFCRARKLDDKFYQKLRGQFPDAVFWQELGEILRQLQKQAAEIYNQSLIELYYEIFIKGRGFANASSVEHYLSDVCYTRAAELFKNAAIASGLRGKVKSNFRLKELKNMKSGLPTTKSDNFPIPLVKQKGGQYAGFEISSHNGDFIIKIPFGRWQVKKEINKYRPWEKFDFEQVRKSPKPISLLLSTQRRKRNKGWSKDEGTEAEIRKVMNGDYQTSYIEVKRGRKIGEKSVWMLNLSIDVPKIDKGVDPSTIGGIDVGVKSPLVCAINNAFSRYSISDNDLFRFNKKMFARRRILLKKNRHKRAGHGAKNKLKPISILTGKSERFRKKLIERWACEIADFFIKNKVGTVQMENLESMKRKEDSYFNIRLRGFWPYAEMQNKIEFKLKQYGIEIRKVAPNNTSKTCSKCGHLNNYFNFEYRKKNKFPHFKCEKCNFKENADYNAALNISNPKLKSTKEKP

SEQ ID NO: 835 - protein, 726 aa, synthetic construct
SEVEFSHEYWMRRALTLAKRARDEREVPVGAVLVLNNRVIGVGWNRAVGLHDPTAHAEIMALRQGGLVMQNYRLIEATLYVTFEPCIMCAGAMIHSRIGRVVFGVRNSKRGAAGSLMNVLNYPGMNHRVEITEGILVDECAALLCDFYRMPRQVFNARKKAQPSINSGGSSDGGSGSETPGTSESATPESSGGSSGGSAKNTITKTLQLRIVRPYNSAEVERIVTDEKNNREKIALEKNKDKVKEACSKHLKMASYCTTQVERNACLFCKARKLDDKFYQKLRGQFPDAVFWQELGGIFRQLQKQAAEIYNQSLIELYYEIFIKGKGITNASRVEHYLSDVCYTRAAELFKNAAIASGLRSKVRSNFRLKELKNMKSGLPTTKSDNFPIPLVKQKGGQYTGFEISSHNSDFIIKIPFGRWQVKEEIDKYRPWEKFDFEQVRKSPKPISLLLSTQRRQKNKGWSEDEGTEAEIRRVMNGDYQTSYIEVKRGSKTGEKSAWMLNLSIDVPKIDKGVDPSIIGGIDVGVKSPLVCAINNAFSRYSISDNDLFRFNKKMFARRRILLKKNRHKRAGHGAKNKLKPISILTEKSKRFRKKLIERWACEIADFFIKNKVGTVQMENLESMKRKEDSYFNIRLRGFWPYAEMQNKIEFKLKQYGIVVRKVAPHNTSKTCSECGHLNNYFNFEYRKKNKFPHFKCEKCNFKENADYNAALNISNPKLKSTKGEP

SEQ ID NO: 836 - protein, 726 aa, synthetic construct
SEVEFSHEYWMRHALTLAKRARVEREVPVGAVLVLNNRVIGEGWNRAIGLHDPTAHAEIMALRQGGLVMQNYRLTDATLYVTFEPCVMCAGAMIHSRIGRVVFGVRNSKRGAAGSLMNVLNYPGMNHCVEITEGILVDECAALLCDFYRMPRQVLNAQKKAQSGISSGGSSGGSSGSEMPGASESVTPKSSAGGSAGSTKNTVTKTLKLRIVRPYNSAEVEKIVADEKNNREKIALEKNKNKVKEACSKHLKVAAYCTTQVERNACLFCKARKLDDKFYQKLRGQFPDAVFWQEIGEIFRQLQKQAAEVYNQSLVELYYEILIKGKGIANASSVEHYLSDVCYTRAAELFKNAAIASGLRNKIKSNFRLKELKNMKSGLPTTKSDNFPIPLVKQKGGQYAGFEISSHNDDFIIKIPFGRWQVKKEIDKYRPWEKFDFEQVRKSPKPISLLLSTQRRKRNKGWSKDEGTEAEIRKVMNGDYQTSYIEVKRGSKTGEKSAWMLNLSIDVPKIDKGVDPSIIGGIDVGVKSPLVCAINNAFSRYSISDNDLFRFNKKMFARRRILLKKNRHKRAGHGAKNKLKPISILTGKSERFRKKLIERWACEIADFFIKNKVGTVQMENLESMKRKEDSYFNIRLRGFWPYAEMQNKIEFKLKQYGIEIRKVAPNNTSKTCSKCGHLNNYFNFEYRKKNKFPHFKCEKCNFKENADYNAALNISNPKLKSTKEEP

SEQ ID NO: 837 - protein, 726 aa, synthetic construct
SEVEFSHEYWMRHALTLAKRARDEREVPVGAVLVLNNRVIGEGWNRAIGLHDPTAHAEIMALRQGGLVMQNYRLTDATLYVTFEPCVMCAGAMIHSRIGRVVFGVRNSKRGAAGSLMNVLNYPGINHCVEITEGILVDECAALLCDFYRMPRQVLNAQKKAQSSISPGGSSGGSSGGETPGTSESATPESSGGSSGGSAKNTITKTLKLRIVRPYNSAEVERIVADEKNNREKIALEKNKDKVKEACSKHLKVASYCTTQVERNACPFCKARKLDDKFYQKLRGQFPDAVFWQELGEILRQLQKQAAEIYNQSLIELYYEIFIKGRGFANASSVEHYLSDVCYTRAAELFKNAAIASGLRGKVKSNFRLKELKNMRSGLPTTKSDNFPIPLVKQKGGQYAGFEISSHNDDFIIKIPFGRWQVKKEIDKYRPWEKFDFEQVRKSPKPISLLLSTRRRKRNKGWSKDEGTEAEIRKVMNGDYQTSYIEVKRGSKIGEKSAWMLNLSIDVPRIDKGVDPSIIGGIDVGVKSPLVCAINNAFGRYSISDNDLFHFNKKMFARRRILLKKNRYKRAGHGAKNKLKPITILTEKSKRFRKKLIERWACEIADFFIKNKVGTVQMENLESMKRKEDSYFNIRLRGFWPYAEMQNRIEFKLKQYGIEIRKVAPNNTSKTCSKCGHLNNYFNFEYRKKNKFPHFKCEKCNFKENADYNAALNISNPKLKSTKEES

SEQ ID NO: 838 - protein, 726 aa, synthetic construct
SEVEFSHEYWMRHALTLAKRARDEREVPVGAILVLNNRVIGEGWNRAIGLHDPTAHAEIMALRQGGLVMQNYRLIDATLYVTFEPCVMCAGAMIHSRIGRVVFGVRNNKHGAAGSLVNVLNYPGMNHCVEITEGILVDECAALLCDFYRMPRQVLNAQKKAQSSISSGGSSGGSSGSETPGASGSVTPKSSGGSSAGSTKDTVTKTLKLRIVRPYNSAEVEKIVADEKNSREKIALEKNKDKVKEACSEHLKVAAYCTTQVERNACLFCKARKLDDGFYQKLRGQFPDAVFWQEIGEIFRQLQKQAAEIYNQSLIELYYEIFIKGKGFANASSVEHYLSDVCYTRAAELFKNAAIASGLRGKVKSNFRLKELKNMKSGLPTTKSDNFPIPLVKQKGGQYTGFEISSHNDDFIIKIPFGRWQVKKETDKYRPWEKFDFEQVRKNPKPISLLLSTQRRKRNKGWSKDEGTEAEIRKVMNGDYQTSYIEVKRGSKIGEKSAWMLNLSIDVPKIDKGVDPSIIGGIDVGVKSPLVCAINNAFSRYSISDNDLFRFNKKMFARRRILLKKSKHKRAGHGAKNKLKPITILTEKSGRFRKKLIERWACEIADFFIKNKVGTVQMENLESMKRKEDSYFNIRLRGFWPYAEMQNKIEFKLKQYGIKIRKVAPNNTSKTCSKCGHLNNYFSFEYRKKNKFPHFKCEKCNFKEDADYNAALNISNPKLKSTKEEP

SEQ ID NO: 839 - protein, 726 aa, synthetic construct
SEVEFSHEYWMRRALTLAKRARDEHEVPVGAVLVLNNRVIGVGWNRAVGLHDPTAHAEIMALRQGGLVMQNYRLIEATLYVTFEPCVMCAGAMIHSRIGRVVFGVRNNKHGAAGSLVNVLNYPGMNHRVEITEGILADECAALLCDFYRMPRQVFNARKKAQSNINPGGSSGGSSGSETPGTSESATPESSGGSSGGSAKNTITKTLKLRIVRPYNSAEVEKIVADEKNNREKIALEKNKDKVKEACSEHLKVAAYCTTQVERSACLFCKARKLDDKFYQKLRGQFPDAVFWQEIGEIFRQLQKQAAEIYNQSLVELYYEIFIKGKGFANASSVEHYLSDVCYTRAAELFKNAAIASGLRGKVKSNFRLKELKNMKSGLPTTKSDNFPIPLVKQKGGQYTGFEISSHNGDFIIKIPFGRWQAKKEIDKYRPWEKFDFEQVRKSPKPISLLLSTQRRKRNKGWSRDEGTEAEIRKVMNGDYQTSYIEVKRGSKIGEKSAWMLNLSIDVPKIDKGVDPSIIGGIDVGVKSPLVCAINNAFSRYSISDNDLFHFNKKMFARRRILLKKNGHKRAGHGAKNKLKPISILTEKSKRFRKKLIERWACEIADFFIKNKVGTVQMEDLESMKRKEDSYFNIRLRGFWPYAEMQNKIEFKLKQYGIEIRKVAPNNTSKTCSKCGHLNNYYNFEYRRKNKFPHFKCEKCNFKEDADYNAALNISNPKLRSTKEEP

SEQ ID NO: 840 - protein, 726 aa, synthetic construct
SEVEFSHEYWMRHALTLAKRARDEREVPVGAVLVLNNRVIGEGWNRAIGLHDPTAHAEIMALRQGGLVMQNYRLTDATLYVTFEPCVMCAGAMIHSRIGRVVFGVRNSKRGAAGSLMNVLNYPGMNHCVEITEGILADECAALLCDFYRMPRQVFSARKKAQSSINPGGSSGGNSGSKTPGTSESATPESSGGSSGGSAKNTITKTLKLRIVRPYNSAEVEKIVADEKNNREKIALEKNKDKVKEACSKHLKVAAYCTTQVERSACLFCKARKLDDKFYQKLRGQFPDAVFWQEIGEIFRQLQKQAAEIYNQSLVELYYEIFIKGKGIANASSVEHYLSDVCYTRAAELFKNAAIASGLRNKIKSNFRLKELRNMKSGLPTTKSDNFPIPLVRQKGGQYTGFEISDHDGDFIIKIPFGRWQVKKEINKHRPWEKFDFEQVRKSPKPISLLLSTQRRKRNKGWSKDEGTEAEIRKVMNGDYQTSYIEVKRGSKIGEKSAWMLNLSIDVPKIDKGVDPSIIGGIDVGVKSPLVCAINNALSRYSISDNDLFHFNKKMFARRRILLRKNRHKRAGHGAKNKLKPITMMTEKSKRFRKKLIERWACEIADFFVKNKVGTVQMENLESMKRKEDSYFNIRLRGLWPYAEMQNKIEFKLKQYGIEIRKVAPNNTSKTCSKCGHLNNYFNFEYRKKNKFPHFKCEKCNFKENADYNAALNISNPKLKSTKEEP

SEQ ID NO: 841 - protein, 726 aa, synthetic construct
SEVGFSHEYWMRHALTLAKRARGEREVPVGAVLVLNNRVIGEGWNRAIGLHDPTAHAEIMALRQGGLVMQNYRLTDATLYVTFEPCVMCAGAMIHSRIGRVVFGARNSKRGAAGSLMNVLSYPGMNHRVEITEGILADECAALLCDFYRMPRRVFNAQKKAQSSINSGGSSGGGSGSETPSTSESTTPESSGGSSGGPAKNTITKTLKLRIVRPYNSAEVEKIVADEKNNREKTALEKNKDKVKEACSKHLKVAAYCTTQVERNACLFCKARKLDDKFYQKLRGQFPDAVFWQEVGEIFRQLQKQAAEIYNQSLIELYYEIFIKGKGFANASSVEHYLSDVCYTRAAELFKNAAIASGLRGKVKSNFRLKELKNMKSGLPTTKSDNFPIPLVKQKGGQYTGFEISNHNGDFIIKIPFGRWQVKKEISRHRPWERFDFEQVRKSPKPISLLLSTQRRKRNKGWGKDEGTEAEIRKVMNGDYQISYIEVKRGSKIGEKSAWMLNLSIDVPKIDKGVDPSIIGGIDVGVKSPLVCAINNALSRYSISDNDLFHFNKKMFARRRILLKKNRHKRAGHGAKNKLKPISVLTEKSGRFRKKLIERWACEIADFFIKNKVGTVQMENLGSMKRKEDSYFNIRLRGFWPYAEMQNKIEFKLKQYGIEIRKVAPNNTSRTCSKCGHLNNYFSFEYRKKNKFPHFKCEKCNFKEDADYNAALNISNPKLKSTKEEP

SEQ ID NO: 842 - protein, 726 aa, synthetic construct
SEVEFSHEYWMRHALTLAKRARDEREVPVGAVLVLNNRVIGEGWNRAIGLHDPTAHAEIMALRQGGLVMQNYRLIDATLYVTFEPCVMCAGAMIHSRIGRVVFGVRNNKHGAAGSLVNVLNYPGMNHRVEITEGILADECAALLCDFYRMPRQVFNARKKAQSSINPGGSSGGSGGSETPGTSESATPESSGGSSGSSAKNTITKTLKLRIVRPYNSAEVEKIVADEKNNREKIALEKNKDKVREACSKHLKVASYCTTQVERNACPFCKARKLDDKFYQKLGGQFPDAVFWQELGEIFRQLQKQAAEIYNQSLVELYYEILIKGKGIANASSVEHYLSDVCYTRAAKLFKNAAIASGLRNKIKSNFRLKELRNMKSGLPTTKSDNFPIPLVKQKGGQYTGFEISSHHDDFIIKIPFGRWQVKKEIDRYRPWEKFDFEQVRKSPKPISLLLSTQRRKRNKGWGKDEGTEAEIRKVMNGDYQTSYIEVRRGSKIGEKSAWMLSLSIDVPKIDKGVDPRIIGGIDVGVKSPLVCAINNAFSRYSISDNDLFHFNKKMFARRRILLKKNRHRRAGHGARNKLKPITVLTEKSKRFRKKLIERWACEIADFFIKNKVGTVQMENLESMKRKEDSYFNIRLRGFWPYAEMQNKIEFKLKQYGIEIRKVAPNNTSKTCSKCGHLNNYFNFEYRRKNKFPHFKCEKCNFKENADYNAALNISNPKLKSTKEEP

SEQ ID NO: 843 - protein, 726 aa, synthetic construct
SEVEFSHEYWMRHALTLAKRARDEREVPVGAVLVLNNRAIGEGWNRAIDLHDPTAHAEIMALRQGGLVMQNYRLTDATLYVTFEPCVMCAGAMIHSRIGRVVFGVRNSKRGAAGSLMNVLNYPGMNHCVEITEGILVDECAALLCDFYRMPRQVLNAQKKAQSSISSGGSSGGSSGSETPGTSESPTPESSGGSPGGSAKNTITKTLQLRIVRPYNSAEVEKIVADEKNNREKIALEKNKDKVKEACSKHLKVASYCTTQVERNACPFCKARKLDDKFYQKLRGQFPDAVFWQELGEILRQLQKQAAEIYNQSLIELYYEIFVKGKGFANASSVEHYLSDVCYTRAAELFKNAAIASGLRGKVKSNFRLRELKSMRSGLPTTKSDNFPIPLVKQKGGQYTGFEISSHNDDFIIKIPFGRWQVKKEIDKYRPWEKFDFEQVRKSPKPISLLLSTQRRKRNKGWSKDEGTEAEIRKVMNGDYQTSYIEVKRGSKVGEKSAWMLSLSIDVPKIDKGVNPSIIGGIDVGVKSPLVCAINNALSRYSVSDNDLFRFNKKMFARRRILLKKNRHKRAGHGAKNKLKPITILTKKSERFRKKLIERWACEIADFFIKNKVGTVQMENLESMKRREDSYFNIRLRGFWPYAEMQNKIEFKLKQYGIEIRKVAPNNTSKTCSKCGHLNNYFNFEYRKKNKFPHFKCEKCNFKENADYNAALNISNPKLKSTKEEP

SEQ ID NO: 844 - protein, 726 aa, synthetic construct
SEVEFSHEYWMRHALTLAKRARDEREVPVGAVLVLNNRVIGEGWNRAIGLHDPTAHAEIMALRQGGLVMQNYRLIDATLYVTFEPCVMCAGAMIHSRIGHVVFGVRNNKHGAAGSLVNVLDYPGMNHRVEITEGILADECAALLCDFYRMPRQVFNARKKAQSSISPGGSSGGSSGSETPGTSESATPESSGGSSGGSAKNTITKTLKLRIVRPYNSAEVEKIVADEKDNRERIALEKNKGKVKEACSKHLKVAAYCTTQVERNACLFCKARKLDDKFYQELRGQFPDAVFWQEVGEIFRQLQKQAAVIYNQSLIELYYEIFIKGKGFANASSVEHYLSDVCYTRAAELFKNAAIASGLRGKVKSNFRLKELKNMKSGLPTTKSDNFPIPLVKQKGGQYTGFEISSHNDDFIIKIPFGRWQVKKEIDKYRPWEKFDFEQVRKSPKPISLLLSTQRRKRNKGWSKDEGTEAEIRKVMNGDYQTSYIEVKRGSKIGEKSAWMLSLSIDVPKIDKGVDPSIIGGIDVGVKSPLVCAINNAFNRYSISDNSLFHFNKKMFARRRILLKKNRHKRAGHGAKNKLKPISILTERSERFRKKLIERWACEIADFFIKNKVGTVQMENLESMKRKEDSYFNIRLRGFWPYAEMQSKIEFKLKQYGIEIRKVAPNNTSKTCSKCGHLNNYFNFEYRKKNKFPHFKCEKCNFKENADYNAALNISNPKLKSTKEEP

SEQ ID NO: 845 - protein, 726 aa, synthetic construct
SEVEFSHEYWMRHALTLAKRARDEREVPVGAVLVLNNRVIGEGWNRAIGLHDPTAHAEIMALRQGGLVMQNYRLTDATLYVTFEPCVMCAGAMIHSRIGRVVFGVRNSKRGAAGSLMNVLNYPGMNHCVEITEGILVDECAALLCDFYRMPRQVLNAQKKAQSSISPGGSSGGSSGSETPGASESVTPKSSGGSSGGSAKNTITKTLKLRIVRPYNSAEVEKIVADEKNNREKIALEKNKGKVKEACSKHLEVAAYCTTQVERNACLFCKARKLDDKFYQKLRGQFPDAVFWQELGEIFRQLQKQAAEIYNQSLIELYYEIFIKGKGFANASSVEHYLSDVCYTRAAELFKNAAIASGLRGKVKSNFRLKELKNMKSGLPTTKSDNFPIPLVKQKGGQYTGFEISSHNDDFIIKIPFGRWQVRKEIDKYRPWEKFNFEQVRKSPKPISLLLSTQRRKRNKGWSKDEGTEAEIRKVMNGDYQTSYIEVKRGSRIGEKSAWMLSLSIDVPKIDRGVDPSIIGGIDVGVKSPLVCAINNALSRYSISDNDLFHFNKKMFARRRILLKKNRHRRAGHGARNKLKPITVLTEKGKRFRKKLIERWACEIANFFIRNKVGTVQMENLESMKRKEDSYFNIRLRGFWPYAEMQNKIEFKLKQYGIEIRRVAPNNTSRTCSKCGHLNSYFNFEYRKKNKFPYFKCEKCNFKENADYNAALNISNPQLKSTKEEP

SEQ ID NO: 846 - protein, 726 aa, synthetic construct
SEVEFSHEYWMRHALTLAKRARDEREVPVGAVLVLNNRVIGEGWNRAIGLHDPTAHAEIMALRQGGLVMQNYRLIDATLYVTFEPCVMCAGAMVHSRIGRVVFGVRNGKRGAAGSLMNVLDYPGMGHRVEVTEGILADECAALLCDFYCMPRQVFNAQKRAQSSINSGGSSGGSSGSETPGTSESATPGSSGGGSSGSAKNTITKTLQLRIVRPYNSAEVEKIVADEKNNREKIALEKNKDKVKEACSKHLKVASYCTTQVERNACPFCKARKLDDKFYQKLRGQFPDAVFWQELGEILRQLQKQAAEIYNQSLIELYYEIFIKGKGFANASSVEHYLSDVCYTRAAELFKNAAIASGLRGKVKSNFRLKELKNMKSGLPTTKSDNFPIPLVKQKGGQYTGFEISNLNSDFIIKIPFGRWQVKKEINKYRPWEKFDFEQVRKSPKPISLLLSTQRRKRNKGWSKDEGTEAEIRKVMNGDYQTSYIEVKRGSKIGEKSAWMLNLSIDVPKIDKGVDPSIIGGIDVGVKSPLVCAINNAFSRYSISDNDLFHFNKKVFARRRILLKKNRHRRAGHGAKNKLKPISILTEKSKRFRKKLIERWACEIADFFIKNKVGTVQMENLESMKRKEDSYFNIRLRGFWPYAEMQNKIEFKLKQYGIEIRKVAPNNTSKTCSKCGHLNNYFNFEYRKKNKFPHFKCEKCNFKENADYNAALNISNPMLKSTKEEP

SEQ ID NO: 847 - protein, 726 aa, synthetic construct
SEVEFSHEYWMRHALTLAKRARDEREVPVGAILVLNNRVIGEGWNRAIGLHDPTAHAEIMALRQGGLVMQNYRLIDATLYVTFEPCVMCAGAMIHSRIGRVVFGVRNNKHGAAGSLVNVLDYPGMNHRVEITEGILADECAALLCDFYRMPRQVFNARKRAQSSINPGGSSGGSSGSETPGTSESATPKSSGGSSGGSAKNTITKTLKLRIVRPYNSAEVEKIVADEKNNREKIALEKNKGKVKEACSKHLEVAAYCTTQVERNACLFCKARKLDDKFYQKLRGQFPDAVFWQEIGEIFRQLQKQAAEIYNQSLIELYYEIFIKGKGFANASSVEHYLSDVCYTRAAELFKNAAIASGLRGKVKSNFRLKELKNMKSGLPTTKSDNFPIPLVKQKGGQYTGFEISSHNDDFIIKIPFGRWQVRKEIDKYRPWEKFNFEQVRKSPKPISLLLSTQRRKRNKGWSKDEGTEAEIRKVMNGDYQTSYIEVKRGSKTGEKSAWMLNLSIDVPKIDKGVDPSIIGGIDVGVKSPLVCAINNAFSRYSISDNDLFRFNKKMFARRRILLKKNRHKRAGHGAKNKLKPISILTGKSERFRKKLIERWACEIADFFIKNKVGTVQMENLESMKRKEDSYFNIRLRGFWPYAEMQNKIEFKLKQYGIEIRKVAPNNTSKTCSKCGHLNNYFNFEYRKMNKFPHFKCEKCNFKENADYNAALNISNPKLKSTKEEP

SEQ ID NO: 848 - protein, 726 aa, synthetic construct
SEVEFSHEFWMRHALTLAKRARDEREVPVGAVLVLNNRVIGEGWNRAIGLHDPTAHAEIMALRQGGLVMQNYRLTDATLYVTFEPCVMCAGAMIHSRIGRVVFGVRNSKRGAAGSLMNVLNYPGMNHCVEITEGILVDECAALLCDFYRMPRQVLNAQKKAQSSISSGGSSGGSSGSETPGASESVTPKSSGGGSAGSTKNTTTKTLKLRIVRPYNSAEVEKIVADEKNNREKIALEKNKGKVKEACSKHLKVATYCTTQVERNACLFCKARKLDDKFYQKLRGQFPDAVFWQEIGEIFRQLQKQAAEIYNQSLIELYYEIFIKGKGFANASSVEHYLSDVCYTRAAELFKNAAIASGLRGKVKSNFRLKELKNMKSGLPTTKSANFPIPLVRQKGGQYTGFEISSHNDDFIIKIPFGRWQVRKEIDKYRPWEKFDFEQVRKSPKPISLLLSTQRRKRNKGWSKDEGTEAEIRKVMNGDYQTSYIEVKRGSKIGEKSAWMLNLSIDVPRIDKGVDPSIIGGIDVGVKSPLVCAINNAFSRYSISDNDLFHFNKKMFARRRILLKKNRHKRAGHGAKNKLKPISILTEKSKRFRKKLIERWACEIADFFIKNKVGTVQMENLESMKRKEDSYFNIRLRGFWPYAEMQNKIEFKLKQYGIEIRKVAPNNTSKTCSKCGHLNNYFNFEYRRKNKFPHFKCEKCNFKEDADYNAALNISNPELKSTKEEP

SEQ ID NO: 849 - protein, 726 aa, synthetic construct
SEVEFSHEYWMRHALTLAKRARDEREVPVGAILVLNNRVIGEGWNRAIGLHDPTAHAEIMALRQGGLVMQNYRLIDATLYVTFEPCVMCAGAMIHSRIGRVVFGVRNNKHGAAGSLVNVLNYPGMNHRVEITEGILADECAALLCDFYRMPRQVFNARKKAQSSINPGGSSGGSSGSETPGTSESPTPESSGGSSGGSAKNTITKTLKLRIVRPYNSAEVEKIVAEEKNNREKIALEKNKDKVKEACSKHLKVAAYCTTQVERNACLFCKARKLDDKFYQKLRGQFPDAVFWQEIGEIFRQLQKQAAEIYNQSLIELYYEIFIKGKGFANASSVEHYLSDVCYTRAAELFKNAAIASGLRGKVKSNFRLKELKNMKSGLPTTKSDNFPIPLVKQKGGQYTGFEISSHNDDFIIKIPFGRWQVKKEIDKYRPWEKFDFEQVRKSPKPISLLLSTQRRKRNKGWSKDEGTEAEIRKVMNGDYQTSYIEVKRGSKIGEKSAWMLNLSIDVPKIDKGVDPSVIGGIDVGVKSPLVCAINNAFSRYSISDNDLFRFNKKMFARRRILLKKNRHKRAGHGAKNKLKPITILTGKSRRFRKKLIERWACEIADFFIKNKVGTVQMESLESMKRKEDSYFNIRLRGFWPYAEMQNKIEFKLKQYGIKIRKVAPNNTSKTCSKCGHLNNYFSFEYRKKNKFPHFKCEKCNFKENADYNAALNISNPKLMSTKEEP

SEQ ID NO: 850 - protein, 726 aa, synthetic construct
SEVEFSHEYWMRHALTLAKRARDEREVPVGAILVLNNRVIGEGWNRAIGLHDPTAHAEIMALRQGGLVMQNYRLTDATLYVTFEPCVMCAGAMIHSRIGRVVFGVRNSKHGAAGSLVNVLNYPGMNHRVEITEGILADECAALLCDFYRMPRQVFNARKKAQSSINPGGSSDGGSGSDTPGTSESATPESSGGGSSGSAKNTITKTLQLRIVRPYNSAEVEKIVADEKNNREKIALEKNKDKVREACSKHLKVASYCTTQVERNACPFCKARKLDDKFYQKLRGQFPDAVFWQELGEILRQLQKQAAEIYNQSLIELYYEIFIKGRGFANAGSVEHYLSDVCYTRAAELFKNAAIASGLRGKVKSNFRLKELKNMKSGLPTTKSDNFPIPLVKQKGGQYTGFEISSHNDDFIIKIPFGRWQVKEEVDKYRPWEKFDFEQVRKNPKPISLLLSTQRRKRNKGWSKDEGTEAEIRKVMNGDYQTSYIEVKRGSKIGEKSAWMLSLSIDVPKIDRGVDPSIIGGIDVGVKSPLVCAINNALSRYSISDNDLFHFNKKMFARRRILLKKNRHRRAGHGARNKLKPITVLTEKSKRFRKKLIERWACEIANFFVKNKVGTVQMENLESMKRKEDSYFNIRLRGLWPYAEMQNKIEFKLKQYGIEVRKVAPNNTSKTCSKCGHLNNYFNFEYRKKNKFPHFKCEKCNFKENADYNAALNISNPKLKSTKEEP

SEQ ID NO: 851 - protein, 726 aa, synthetic construct
SEVEFSHEYWMRHALTLAKRARDKHEVPVGAVLVLDNRVIGEGWNRATGQNDPTAHAEIMALRQGGLVMQNHRLIDATLYVTFEPCVMCAGAMIHSRIGRVVIGVRNSKRGAAGSLMNVLNHPGMNHRVEITEGILADECAALLCDFYRMPRQVFNAQEKAQSSINSGGSSGGSSGSETPGTSESATPGSSGGSSAGSTKDTITKTLKLRIVRPYNSAEVEKIVADEKNNREKIALEKNKGKVKEACSKHLKVAAYCTTQVERNACLFCKARRLDDKFYQKLRGQFPDAVFWQEIGEVFRQLQKQAAEIYNQSLVELYYEIFIKGKGIANASSVEHYLSDVCYTRAAELFKNAAIASGLRNKIKSNFRLKELRNMKSGLPTTKSDNFPIPLVRQKGGQYTGFEISNHNGDFIIKIPFGRWQVKKEISKHRPWEKFDFEQVRKSPKPISLLLSTQRRKRNKGWGKDEGTEAEIRKVMNGDYQTSYIEVKRGSKIGEKSAWMLNLSIDVPKIDKGVDPSIIGGIDVGVKSPLVCAINNALSRYSISDNDLFHFNKKMFARRRILLRKNRHKRAGHGARNKLKPITIMTEKSKRFRKKLIERWACEIADFFVKNKVGTVQMESLESMKRKEDSYFNIRLRGFWPYAELQNKIEFKLKQYGIVVRKVAPNNTSRTCSKCGHLNNYFNFEYRKKNKFPHFKCEKCNFKENADYNAALNISNPKLKSTKEEP

SEQ ID NO: 852 - protein, 726 aa, synthetic construct
SEVGFSHEYWMRHALTLAKRARDEREVPVGAVLVLNNRVIGEGWNRAIGLHDPTAHAEIMALRQGGLVMQNYRLTDATLYVTFEPCVMCAGAMIHSRIGRVVFGVRNSKRGAAGSLMNVLNYPGMNHCVEITEGILVDECAALLCDFYRMPRQVLNAQKKAQSSISSGGSSGGSSCSETPGASESVTPKSSGGSSAGSTKNTITKTLKLRIVRPYNSAEVEKIVADEKNNREKIALEKNKDKVKEACSKHLKVASYCTTQVERNACPFCKARKLDDKFYQKLRGQFPDAVFWQELGEIFRQLQKQAAEIYNQSLIELYYEIFIKGKGFANASSVEHYLSDVCYTRAAELFKNAAIASGLRGKVKSNFRLKELKNMKSGLPTTKSDNFPIPLVKQKGGQYTGFEISSHNDDFIIKIPFGRWQVKKEINKFRPWEKFDFEQVRKSPKPISLLLSTQRRKRNKGWSRDEGTEAEIRKVMNGDYQTSYIEVKRGSKIGEKSAWMLNLSIDVPKIDKGVDPSIIGGIDVGVKSPLVCAINNSSSRYSICDNDLFRFNKKMFARRRILLKKNRHKRAGHGAKNKLKPITILTKKSERFRKKLIERWVCEVADFFIKNKVGTVQMENLESMKRKEDSYFNIRLRGFWPYAEMQNRIELKLKQYGIEIRRVAPNNTSRTCSKCGHLNNYFNFEYRKKSKFPHFKCEKCNFREDADYNAALNISNPKLKSTKEEP

SEQ ID NO: 853 - protein, 726 aa, synthetic construct
SEVEFSHEYWMRHALTLARRARDEREVPVGAILVLNNRVIGEGWNRAIGLHDPTAHAEIMALRQGGLVMQNYRLVDATLYVTFEPCVMCAGAMIHSRISRVVFGVRNNKHGAAGSLMNVLNYPGMNHRVEITEGILEDECAALLCDFYRMPRQVFNARKKAQSSINSGGSSGGSSGSETPGTSESATPESSGGSSGGSAKNTITKTLKLRIVRPYNSAEVEKIVADEKNNREKIALEKNKDKVKEACSEHLKVAAYCTTQVERNACLFCRARKLDDKFYQKLRGQFPDAVFWQEIGEIFRQLQKQAAEVYNQSLIELYYEIFIKGKGFANASSVEHYLSDVCYTRAAELFKNAAIASGLRGKVKGNFRLKELKNMKSGLPTTKSDNFPIPLVKQKGGQYTGFEISSHNDDFIIKIPFGRWQVKKEIDKYRPWEKFDFEQVRKSPKPISLLLSTQRRKRNKGWSKDEGTEAEIRKVMNGDYQTSYIEVERGSKIGEKSAWMLNLSIDVPKIDKGVDPSIIGGIDVGVKSPLVCAINNAFSRYSIGDNDLFHYNKKMFARRRILLKKNRHKRAGHGAKNKLKPISILTEKSKRFRKKLIERWACEIADFFIKNKVGIVQIENLESMKRREDSYFNIRLRGFWPYAEMQNKIEFKLKQYGIEIRKVAPNNTSKTCSKCGHLNSYFNFEYRKKNKFPHFKCEKCNFKENADYNAALNISNPKLKCTKEKP

SEQ ID NO: 854 - protein, 726 aa, synthetic construct
SEVGFSHEYWMRHALTLAKRARDEREVPVGAVLVLNNRVIGEGWNRAIGLHDPTAHAEIMALRQGGQVMQNYRLVDATLYVTFEPCVLCAGAMVHSRIGHVVFGVRNSKRGAAGSLMNVLNHPGMSHRVEVTEGILADECAALLCDFYRMPRQVFNAQKKARSNINSGGSSGGSSGSEAPGTSESATPKSSGGSSAGSTKNTITKTLKLRIVRPYNSAEVEKIVADEKNSREKIALERNKDKVREACSEHLKVAAYCTTQVERNACLFCKARKLDDGFYQKLRGQFPDAVFWQEIGEIFRQLQKQAAEIYNQSLIELYYEIFIKGKGFANASSVEHYLSDVCYTRAAELFKNAAIASGLRGKVKSNFRLKELKNMKSGLPTTKSDNFPIPLVRQKGGQYTGFEISCHNDDFIIKIPFGRWQAKEEIDKYRPWEKFDFEQVRKSPKPISLLLSTQRRKRNKGWSKDEGTEAEIRKVMNGDYQTSYIEVKRGSKIGEKSAWMLNLSIDVPKIDKGVDPSIIGGIDVGVKSPLVCAINNAFSRYSIGDNDLFHFNKKMFARRRILLKKNKHRRAGHGVKNKLKPISILTEKSKRFRKKLIERWACEIADFFIKNKVGTVQMENLESMKRKEDSYFNIRLRGFWPYAEMQNKIEFKLKQYGIEIRKVAPNNTSKICSKCGHLNNYFNFEYRRKNKFPHFKCEKCNFKENADYNAALNVSNPKLKSTKEEP

SEQ ID NO: 855 - protein, 726 aa, synthetic construct
GEVEFSHEYWMRHALTLAKRARDEREVPVGAVLVLNNRVIGEGWNRAIGLHDPTAHAEIMALRQGGLVMQNYRLVDATLYVTFEPCVLCAGAMVHSRIGRVVFGVRNSKRGAAGSLMNVLNYPGMNHRVEITEGILADECAALLCDFYRMPRQVLNTQKKAQSSINPGGSSGGSSGSETPGTSESATPESSGGSSGSSAKNTITKTLKLRIVRPYNSAEVEKIVADEKNNREKIALEKNKDKVKEACSKHLKVAAYCTTQVERNACLFCKARRLDDKFYQKLRGQFPDAVFWQEIGEIFRQLQKQAAEVYNQSLVELYYEILIKGKGIANASSVEHYLSDVCYTRAAELFKNAAIASGLRNKIKSNFRLKELRNMKSGLPTTKSDNFPIPLVKQKGGQYTGFEISNHNSDFIIKIPFGRWQAKKEIDKYRPWEKFDFEQVRKSPKPISLLLSTQRRKRNRGWSKDEGTEAEIRKVMNGDYQTSYIEVKRGSKIGEKSAWMLNLSIDVPKIDKGVDPSIIGGIDVGVKSPLVCAINNAFSRYSISDNDLFRFNKKMFARRRILLGKNRHKRAGHGVKNKLKPITILTEKSGRFRKKLIERWACEIADFFVKNKVGTVQMENLESMKRKEDSYFNIRLRGFWPYAEMQNKIEFKLKQYGIEIRKVAPNNTSKTCSKCGHLNNYFSFEYRKKNKFPHFKCEKCNFKEDADYNAALNISNPKLKSTKEEP

SEQ ID NO: 856 - protein, 726 aa, synthetic construct
SEVEFSHEYWMRHALTLAKRARDEREVPVGAVLVLNNRVIGEGWNRTTGLHDPTAHAEIMALRQGGLVMQNHRLVDATLYVTFEPCVMCAGAMIHSRIGRVVFGVRNSKRGAAGSLTNVLNYPGMNHRVEITEGILVDECAALLCDFYRMPRQVFNAQKKARSTINSGGSSGGSSGSVTPGTSESAAPESSGGSFGGSAKNTITKTLQLRIVRPYNSAEVEKIVADEKNNRERIALEKNKDKVKEACSKHLKVAAYCTTQVERNACLFCKARRLDDKFYQKLRGQFPDAVFWQELGEILRQLQKQAAEIYNQSLIELYYEIFIKGKGFANASSVEHYLSDVCYTRAAELFKNAAIASGLRGKVKSNFRLKELKNMKSGLPTTKSDNFPIPLVKQKGGQYTGFEVSNHNSDFIIKIPFGRWQEKEEIDKYRPWEKFDFEQVRRSPKPISLLLSTQRRKKNKGWSKDEGTEAEIRRVMNGDYQTSYIEVRRGSKTGEKSAWMLNLSIDVPKIDKGVDPSIIGGIDVGVKSPLVCAINNAFSRYSISDNDLFRFNKKMFARRRILLKKNRHKRAGHGAKNKLKPITILTEKSVRFRKKLIERWACEIADFFIRNKVGTVQMENLESMKRKEDSYFNIRLRGFWPYAEMQNKIEFKLKQYGIEIRKVAPNNTSKTCSRCGHLNNYFNFEYRKKNKFPHFKCEKCNFKENADYNAALNISNPKLKSTKEEP

SEQ ID NO: 857 - protein, 726 aa, synthetic construct
SEVEFSHEYWMRHALTLAKRARDEREVPVGAVLVLNNRVIGEGWNRAIGLHDPTAHAEIMALRQGGLVMRNYRLTDATLYVTFEPCVMCAGAMIHSRIGRVVFGVRNSKRGAAGSLMNVLNYPGMNHCVEITEGILVDECAALLCDFYRMPRQVLNAQKKAQSSINPSGSSGGSSGSVTPGISESATPESSGGGFGGSAKNTITKTLQLRIVRPYNSAEVEKIVADEKNNREKIALEKNKDKVKEACSEHLKVAAYCTIQVERNACLFCKARKLDDKFYQKLRGQFPDAVFWQELGGIFRQLQKQAAEIYNQSLIELYYEIFIKGKGLANASSVEHYLSDVCYTRAAELFKNAAIASGLRGKVKSNFKLKELKNMKSGLPTTKSDNFPIPLVKQKGGQYTGFEISSHNDDFIIKIPFGRWQVRKEIDKYRPWEKFNFEQVRKSPKPISLLLSTQRRKRNKGWSKDEGTEAEIRKVMNGDYQTSYIEVKRGSKIGEKSAWMLSLSIDVPKIDKGVDPSIIGGIDVGVKSPLVCAIYNAFSRYSISDNDLFHFNKKMFARRRILLKKNRRKRAGHGAKNKLKPISILTEKSKRFRKKLIERWACEIADFFIKNKVGTVQMENLESMKRKEDSYFNIRLRGFWPYAEMQNKIEFKLKQYGIEIRKVAPNNTSKTCSKCGHLNNYFNFEYRKRNKFPHFKCKKCNFKENADYNAALNISNPKLKSPKEEP

SEQ ID NO: 858 - protein, 726 aa, synthetic construct
SEVEFSHEYWMRHALTLAKRARDEREVPVGAVLVLNNRVIGEGWNRAIGLHDPTAHAEIMALRQGGLAMQNYRLVDATLYVTFEPCVLCAGAMVHSRIGRVVFGVRNSKRGAAGSLMNVLNHPGMNHRVEITGGILADECAALLCDFYRMPRQVFNAQKKARSNINSGGSSGGSSGSETLGTSESATPESSGGSPGGSAKNTITKTLKLRIVRPYNSAEVEKIVADEKNNREKIALEKNKDKVKEACSEHLKVAAYCTTQVERNACLFCKARKLDDKFYQRLRGQFPDAVFWQELGEIFRQLQKQAAEIYNQSLIELYYEIFIKGKGFANASSVEHYLSDVCYTRAAELFKNAAIASGLRGKVKSNFRLKELKNMKSGLPTTKSDNFPIPLVKQKGGQYTGFEISSHNDDFIIKIPFGRWQVKKEIDKYRPWEKFDFEQVRRSPKPISLLLSTQRRRRNKGWSKDEGTEAEIRKVMNGDYQASYIEVKRGSKIGEKSAWMLNLSIDVPKIDKGVDPSIIGGIDVGVKSPLVCAINNAFSRYSISDNDLFHFNKKVFARRRILLKKNRHRRAGHGAKNKLKPITILTEKSKRFRKKLIERWACEIADFFIKNKVGTVQMENLESMKRKEDSYFNIRLRGFWPYAEMQNKIEFKLKQYGIKIRKVAPNNTSRTCSKCGHLNNYFNFEYRKKNKFPHFKCEKCNFKENADYNAALNISNPKLKSTKEEP

SEQ ID NO: 859 - protein, 726 aa, synthetic construct
SEVEFSHEYWMRHALTLAKRARDEREVPVGAVLVLNNRVIGEGWNRAIGLHDPTAHAEIMALRQGGLVMQNYRLTDATLYVTFEPCVMCAGAMIHSRIGRVVFGVRNSKRGAAGSLMNVLNYPDMNHCVEITEGILVDECAALLCDFYRMPRQVLNAQKKAQSSISSGGSSGGSSGSETPGASESATPKSSGGSSASSTKNTITKTLKLRIVRPYNSAVVEKIVADEKNSREKIALEKNKDKVKEACSEHLKVAAYCTTQVERNACLFCKARKLDDGFYQKLRGQFPDAVFWQEIGEIFRQLQKQAAEIYNQSLIELYYEIFIKGKGFANASSVEHYLSDVCYTRAAELFKNAAIASGLRGKVKSNFRLKELKNMKSGLPTTKSDNFPIPLVKQKGGQYTGFEISNHNSDFIIKIPFGRWQVKKEIDKYRPWEKFDFEQVRKSPKPISLLLSTQRRKRNRGWSKDEGTEAEIKKVMNGDYQTSYIEVKRGSKTGEKSAWMLNLSIDVPKIDKGVDPCIIGGIDVGVKSPLVCAINNASSRYSISDNDLFHFNKKMFARRRILLKKNGHKRAGHGTKNKLKPITIMTEKSKRFRKKLIERWACEIADFFIKNKVGTVQMENLESMKRKEDSYFNIRLRGFWPYAELQNKIEFKLKQYGIVVRKVAPNNTSKTCSKCGHLNNYFNFEYRKKNKFPHFKCEKCNFKENADYNAALNISNPKLKSTKGGP

SEQ ID NO: 860 - protein, 726 aa, synthetic construct
SEVEFSHEYWMRHALTLAKRARDEREVPVGAVLVLNNRVIGEGWNRAIGLHDPTAHAEIMALRQGGLAMQNYRLVDATLYVTFEPCVLCAGAMVHSRIGRVVFGVRNSKRGAAGSLMNVLNHPGMNHRVEITGGILADECAALLCDFYRMPRRVFNAQKKARSNINSGGSSGGSSGSEAPGTSESATPESSGGSSGGSAKNTITKTLQLRIVRPYNSAEVEKIVADEKNNREKIALEKNKDKVKEACSQHLKMASYCTTQVERNACLFCKARKLDDKFYQKLRGQFPDAVFWQEIGEIFRQLQKQAAEIYNQSLIELYYEIFIKGKGFANASSVEHYLSDVCYTRAAELFKNAAIASGLRNKIKSNFRLKELRNMKSGLPTTKSDNFPIPLVRQKGGQYTGFEISNHDGDFIIKIPFGRWQVKKEINKHRPWEKFDFEQVRKSPKPISLLLSTQRRKRNKGWSKDEGTEAEIRKVMNGDYQTSYIEVKRGSKIGEKGAWMLNLSIDVPKIDKSVDPSIIGGIDVGVKSPLVCAINNALSRYSISDNDLFHFNKKMFARRRILLRKNRHKRAGHGARNKLKPITVLTEKSERFRKKLIERWACEIANFFIKNKVGTVQMEDLESMKRREDSYFNIRLRGFWPYAEMQSKIEFKLKQYGIKIRKVAPNNTSKTCSKCGHLNNYFSFEFRKKNKFPHFKCEKCNYKENADYNAALNISNPKLKSTKEEP

SEQ ID NO: 861 - protein, 726 aa, synthetic construct
SEVEFSHEYWMRHALTLAKRARDEREVPVGAILVLNNRVIGEGWNRAIGLHDPTAHAEIMALRQGGLVMQNYRLIDATLYVTFEPCVMCAGAMIHSRIGRVVFGVRNSKHGAAGSLVNVLNYPGMNHRVEITEGILADECAALLCNFYRMPRQVFNVRKKAQSSINPGGSSGGSSGSETPGTSESATPESSGGSSGGSAKNTITKTLKLRIVRPYNSAEVEKIVADEKNNREKIALEKNKDKVKEACSKHLKVAAYCTTQVERNACLFCKARRLDDKFYQKLRGQFPDAVFWQEIGEIFRQLQKQAAEIYNRSLIELYYEIFIKGKGIANASRVEHYLSDVCYTRAAELFKNAAIASGLRNRIKSNFRLKELKNMKSGLPTTKSDNFPIPLVKQKGGQYTGFEISNHNSDFIIKIPFGRWQAKKEIDKYRPWEKFDFEQVRKGPKPISLLLSTQRRKRNKGWSKDEGTEAEIRKVMNGNYQTSYIEVKRGSKIGEKNAWMLSLSIDVPKIDKGVDPSIIGGIDVGVKSPLVCAINNALSRYSISDNDLFHFNKKMFARRRILLKKNRHKRAGHGARNKLRPITVLTEKSERFRKKLIERWACEIANFFIKNRVGTVQMENLESMKRKEDSYFNIRLRGFWPYAEMQNKIEFKLKQYGIEVRKVAPNNTSKTCSKCGHLNNYFNFEYRKKNKFPHFKCEKCNFKENADYNAALNISSPKLKSTREEP

SEQ ID NO: 862 - protein, 726 aa, synthetic construct
SEVEFSHEYWMRHALTLAKRARDGREVPVGAVLVLNNRVIGEGWNRAIGLHDPTAHAEIMALRQGGLVMQNYRLIDATLYVTFEPCVMCAGALVHSRIGRVVFGVRNSKRGAAGSLMNVLDYPGMGHRVEITEGILADECAALLCDFYCMPRQVFNAQKKAQSSINPGGSSGGSSGSETPGTSESATPESSGGSSGGSAKNTITKTLKLRIVRPYNSAEVEKIVADEKNNREKIALEKNKGKVKEACSKHLEVAAYCTTQVERNACLFCKARKLDDKFYQKLRGQFPDAVFWQELGEIFRQLQKQAAEIYNQSLIELYYEIFIKGKGFANASSVEHYLSDVCYTRAAELFKNAAIASGLRGKVKSNFRLKELKNMKSGLPTTKSDNFPIPLVKQKGGQCTGFEISSHNDDFIIKIPFGRWQAKEEIDKYRPWEKFDFEQVRKSPKPISLLLSTQRRKRNKGWSKDEGTEAEIRKVMNGGYQTSYIEVKRGSKIGEKSAWMLNLSIDVPKIDKGVDPSIIGGIDVGVKSPLVCAINNAFSRYSISDNDLFHFNKKMFARRRILLKKNRHKRAGHGAKNKLKPISILTEKSKRFRKKLIERWACEIANFFIKNKVGTVQMENLESMKRKEDSYFNIRLRGFWPYAEMQNKIEFKLKQYGITIRRVAPNNTSKTCSKCGHLNNYFSFEYRKRNKFPHFKCEKCNFKEDADYNAALNISNPKLKSTKEEP

SEQ ID NO: 863 - protein, 726 aa, synthetic construct
SEVEFSHEYWMRRALTLAKRARDEREVPVGAVLVLNNRVIGVGWNRAVGLHDPTAHAEIMALRQGGLVMQNYRLVEATLYVTFEPCIMCAGAMIHSRIGRVVFGVRNSKRGAAGSLMNVLNYPGMNHRVEITEGILADECAALLCDYYRMPHQVFNARKKAQSSINSGGSSDGGSGSETPGTSESATPESSGGSSGGSAKNTITKTLKLRIVRPYNSAEVEKIVADEKNNREKIALEKNKDKVKEACSEHLKVAAYCTTQVERSACLFCKARKLDDKFYQKLRGQFPDAVFWQEIGEIFRQLQKQAAEIYNQSLIELYYEIFIKGKGFANASSVEHYLSDVCYTRAAELFKNAAIASGLRGKVKSNFRLKELKNMKSGLPTTKSDNFPIPLVKQKGGQYTGFEISSHNDDFIIKIPFGRWQVKKEIDKYRPWEKFDFEQVRKSPKPISLLLSTQRRKRNKGWSRDEGTEAEIRKVMNGDYQTSYIEVKRGSKVGEKSAWMLSLSIDVPKIDKGVDPSIVGGIDVGVKSPLVCAINNAFGRYSISDNDLFHFNKKMFARRRILLKKSKHKRAGHGAKNKMKPITILTEKSGRFRKKLIERWACEIADFFIKNKVGTVQMENLESMKRKEDSYFNIRLRGFWPYAEMQNKIEVKLKQYGIEIRKVAPNNTSKTCSKCGHLNSYFNFEYRKKNKFPHFKCEKCNFKEDADYNAALNISNPKLKSTKEEP

SEQ ID NO: 864 - protein, 726 aa, synthetic construct
SEVEFSHEYWMRHALTLAKRARDEREVPVGAILVLNNRVIGEGWNRAIGLHDPTAHAEIMALRQGGLVTQNYRLTDATLYVTFEPCVMCAGAMIHSRIGRVVFGVRNSKRGAAGSLMNVLNYPGMNHCVEITEGILVDECAALLCDFYRMPRQVLNAQKKAQSSISSGGSSGGSSGSEKPSASESVAPKSSVGSSAGSTKNTITKTLKLRIVRPYNSAEVEKIVADEKDNREKIALERNKGKVKEACSKHLEVAAYCTTQVERNACLFCKARKLDDKFYQKLRGQFPDAVFWQELGEILRQLQKQAAEIYNQSLIELYYEIFIKGKGFANASSVEHHLSDVCYTRAAELFKNAAIASGLRGKVKSNFRLKELKNMKSGLPTTKSDNFPIPLVKQKGGQYTGFEISSHNDDFIIKIPFGRWQVKKEIDKYRPWEKFDFEQVRKSPKPISLLLSIQRRKRSKGWSKDEGTEAEIRKVMNGDYQTSYIEVKRGSKIGEKSAWMLNLSIDVPKIDKGVDPSIIGGIDVGVKSPLVCAVNNAFSRYSISDNELFHFNKKMFARRRILLKKNRHKRAGHGAKNKLKPISTLTERSKRFRKKLIERWACEIADFFIKNKVGTVQMENLESMKRKEDSYFNIRLRGFWPYAEMQNKIEFKLKQYGIEIRKVAPNNTSKTCSKCGHLNNYFNFEYRKKNKFPHFKCEKCNFKENADYNAALNISNPKLKSTKKEP

SEQ ID NO: 865 - protein, 726 aa, synthetic construct
SEVEFSHEYWMRHALTLAKRARDEREVPVGAVLVLNNRVIGGGWNRAIGLHDPTAHAEIMALRQGGLVMQSCRLVDATLYVTFEPCVMCAGAMIHSRIGRVVFGVRNSKRGAAGSLMNVLNYPGMNHRVEITEGILAGECAALLCDFYRMPRQVFNAQKKAQSTINSGGSSGGSSSSETPGTSGSATPEGSGGSSGSSAKNTITKTLKLRIVRPYNSAEVEKIVADEKNNREKIALEKNKDKVKEACSKHLKVAAYCTTQVERNACLFCKARRLDDKFYQKLRGQFPDAVFWQEIGEIFRQLQKQAAEVYNQSLVELYYEILIKGKGIANASSVEHYLSDVCYTRAAELFKNAAIASGLRNKIKSNFRLKELRNMKSGLPTTKSDNFPIPLVRQKGGQYTGFEISNHDGDFIIKIPFGRWQVKKEINKHRPWEKFDFEQVRKSPKPISLLLSTQRRKRNKGWSKDEGTEAEIRKVMNGDYQTSYIEVKRGSKIGEKSAWMLNLSIDVPKIDKGVDPSIIGGIDVGVKSPLVCAINNAFGRYSISDNDLFRFNKRMFARRRILLGKNRHKRAGHGVKNKLKPITILTEKSGRFRKKLIERWACEIADFFVKNKVGTVQMENLESMKRKEDSYFNIRLRGFWPYAEMQNKIEFKLKQYGIEIRKVAPNNTSKTCSKCGHLNSYFDFEYRKKNKFPHFKCEKCNFKENADYNAALNISNPKLKSTKEEP

SEQ ID NO: 866 - protein, 726 aa, synthetic construct
SEVEFSHEYWMRHALTLAKRARDEREVPVGAVLVLNNRVIGEGWNRTTGLHDPTAHAEIMALRQGGLVMRNYRLTDATLYVTFEPCVMCAGAMIHSRIGRVVFGVRNSKRGAAGSLVNVLNYPGMNHRVEITEGILADECAALLCDFYRMPRQVFNARKKAQSTINSGSSSGGSSGSETPGTSESPTPESSGGIPGGSAKNTITKTLKLRIVRPYNSAEVEKIVADEKNNREKIALEKNKDKVKEACSKHLKVAAYCTTQVERNACLFCKARKLDDKFYQKLRGQFPDAVFWQEIGEIFRQLQKQAAEIYNQSLIELYYEIFIKGKGFANASSVEHYLSDVCYTRAAELFKNAAIASGLRGKVKSNFRLKELKNMKSGLPTTKSDNFPIPLVKQKGGQYTGFEIGSHNDDFIIKIPFGRWQVKEEIDKYRPWEKFDFEQVRKNPKPISLLLSTQRRKRNKGWSKDEGTEAEIRKVMNGDYQTSYIEVKRGSKIGEKSAWMLNLSIDVPKIDKGVDPSIIGGIDVGVKSPLVCAINNAFSRYSISDNDLFRFNKKMFARRRILLKKNRHKRAGHGAKNKLKPITILTEKSRRFRKKLIERWACEIADFFIKNKVGTVQMESLESMKRKEDSYFNIRLRGFWPYAEMQNKIEFKLKQYGIKIRKVAPNNTSRTCSMCGHLNNYFSFEYRKKNKFPHFKCEKCNFKENADYNAALNISNPKLMSTKEGP

SEQ ID NO: 867 - protein, 726 aa, synthetic construct
SEVEFSHEYWMRHALTLAKRARDEREVPVGAILVLNNRVIGEGWNRAIGLHDPTAHAEIMALRQGGLVMQNYRLIDATLYVTFEPCVMCAGAMIHSRIGRVVFGVRNNKHGAAGSLVNVLNYPGMNHRVEITEGILADECAALLCDFYRMPRQVFNARKKAQSSINPGGSSGGSSGSETPGTSESATPESSGGGSSGSAKNTITKTLQLRIVRPYNSAEVEKIVADEKNNREKIALEKNKDKVKEACSKHLKVASYCTTQVERSACPFCKARKLDDKFYQKLGGQFPDAVFWQELGEILRQLQKQAAEIYNQSLIELYYEIFIKGRGFANASSVEHYLSDVCYTRAAELFKNAAIASGLRGKVKSNFRLKELKNMKSGLPTTKSDNFPIPLVKQKGGQYTGFEISSHNDDFIIKIPFGRWQVKKEINKYRPWEKFDFEQVRKSPKPISLLLSTQRRKRNKGWSKDEGTEAEIRKVMNGDYQTSYIEVRRGSKIGERSAWMLNLSIDVPKIDKGVDPSTIGGIDVGVKSPLVCAINNAFSRYSISDNDLFRFNKKMFARRRILLGKNRHKRAGHGVKNKLKPITILTEKSGRFRKKLIERWACEIADFFVKNKVGTVQMENLESMKRKEDSYFNIRLRGFWPYAEMQNKIEFKLKQYGIKVRKVAPNNTSKTCSKCGHLNNYFSFEYRKKNKFPHFKCEKCDFKENADYNAALNISNPKLKSTKEEP

SEQ ID NO: 868 - protein, 726 aa, synthetic construct
SEVEFSHEYWMRHALTLAKRARDEREVPVGAILVLNNRVIGEGWNRAIGLHDPTAHAEIMALRQGGLVMQNYRLIDATLYVTFEPCAMCAGAMVHSRIGRVVFGVRNSKRGAAGSLMNVLNYPGMDHRVEITGGILADECAALLCDFYRMPRRVFNAQKKAHSSINSGGSSGGSSGSVTPGTSESATPESSGGGFGDSAKNTITKTLQLRIVRPYNSAEVEKIVADEKNNREKIALEKNKDKVKEACSKHLKVASYCTTQVERNACLFCKARKLDDKFYQKLRGQFPDAVFWQELGEIFRQLQKQAAEIYNQSLIELYYEIFIKGKGLANASSVEHYLSDVCYTRAAELFKNAAIASGLRGKVKSNFKLKELKSMKSGLPSTKSDNFPIPLVKQKGGQYTGFEISSHNDDLIIKIPFGRWQVKREIDKYRPWEKFDFEQVRKSPKPISLLLSTQRRKRNKGWSKDEGTEAEIRKVMNGDYQTSYIEVKRGSKVGEKSAWMLNLSIDVPKIDKGVDPSIIGGVDVGVKSPLVCAINNAFSRYSISDNDLFRFNKRMFARRRILLKKNRHKRAGHGTKNKLKPITILTEKSGRFRKKLIERWACEIANFFIKNKVGTVQMENLESMKRKEDSYFNIRLRGFWPYAEMQNKIEFKLKQYGIKIRKVAPNNTSKTCSKCGHLNNYFSFEYRKKNKFPHFKCEKCNFKEDADYNAALNISNPELKSTKEEP

SEQ ID NO: 869 - protein, 726 aa, synthetic construct
SEVEFSHEYWMRHALTLAKRARDEREVPVGAVLVLNNRVIGEGWNRAIGLHDPTAHAEVMALRQGGLVMQNYRLTDATLYVTFEPCVMCAGAMIHSRIGRVVFGVRNSKRGAAGSLMNVLNYPGMNHCVEITEGILVDECAALLCDFYRMPRQVLNAQKKAQSSISPGDSSGGSSGSETPGASGSVTPKSSGGSSAGSTKDTITKTLKLRIVRPYNSAEVEKIVADEKNSREKIALEKNKDKVKEACSKHLKVASYCTTQVERNACLFCKARKLDDKFYQKLRGQFPDAVFWQEVGGIFRQLQRQAAEIYNQSLIELYYEIFIKGKGFANASSVEHYLSDVCYTRAAELFKNAAIASGLRGKVKSNFRLKELKNMKSGLPTTKSDNFPIPLVRQKGGQYTGFEISSHNDDFIIKIPFGRWQVKKEIDKYRPWEKFDFEQVRKSPKPISLLLSTQRRKRNKGWSKDEGTEAEIRKVMNGDYQISYIEVKRGSKIGEKSAWTLNLSVDVPKIDKGVDPSIIGGIDVGVKSPLVCAINNAFSRYSISDNDLFRFNKKMFARRRILLKKNRHKRAGHGAKNKLKPISILTGKSERFRKKLIERWACEIADFFIKNKVGTVQMENLESMKRREDSYFNIRLRGFWPYAEMQNKIEFKLRQYGIEIRKVAPNNTSKTCSKCGHLNNYFDFEYRKKNKFPHFKCEKCNFKENADYNAALNISNPKLRSTKEEP

SEQ ID NO: 870 - protein, 726 aa, synthetic construct
SEVEFSHEYWMRHALTLAKRARDEREVPVGAVLVLNNRVIGEGWNRTTGLHDPTAHAEIMALRQGGLVMQNHRLVDATLYVTFEPCVMCAGAMIHSRIGRVVYGIRNSKRGAAGSLTNVLDYPGMSHRVEITEGILADECAALLCDFYRMPRQVFNAQKKAQSNINPGGSSGGSSGSETPGTSKSATPGSSGGSSGGSAKNTITKTLKLRIVRPYNSAEVEKIVADEKNNREKIALEKNKDKVKEACSEHLKVAAYCTTQVERNACLFCKARRLDDKFYQKLRGLFPDAVFWQELGEIFRQLQKQAAEIYNQSLIELYYEIFIKGKGITNASRVEHYLSDVCYTRAAELFKNAAIASGLRSKVRSNFRLKELKNMKSGLPTTKSDNFPIPLVKQKGGQYTGFEISSHNSDFIIKIPFGRWQAKKEIDKYRPWEKFDFEQVRKSPKPISLLLSTQRRKKNKGWSKDEGTEAEIRKVMNGDYQTSYIEVKRGSKIGEKSAWMLNLSIDVPKIDKGVDPSIIGGIDVGVKSPLVCAINNAFSRYSISDNELFHFNKKMFARRRILLKKNRHKRAGHGAKNKLKPIAIMTEKSKRFRKKLIERWACEIADFFIKNKVGTVQMEDLESMKRKEDSYFNIRLRGFWPYAEMQNKIEFKLKQYGIVVRKVAPNNTSKTCSKCGHLNNYFNFEYRKKNKFPHFKCEKCNFKEDADYNAALNISNPKLKSTKGEP

SEQ ID NO: 871 - protein, 726 aa, synthetic construct
SEVEFSHEYWMRHALTLAKRARDEREVPVGAVLVLNNRVIGEGWNRAIGLHDPTAHAEVMALRQGGLVMQNYRLTDATLYVTFEPCVMCAGAMIHSRIGRVVFGVRNSKRGAAGSLMNVLNYPGMNHCVEITEGILADECAALLCDYYRMPRRVFNARKKAQSSINSGGSSDSGSGSETPGTSESATPESSSGSSGGSAKNTITKTLKLRIVRPYNSAEVERIVADEKNNREKIALEKNKDKVKEACSKHLKVAAYCTTQVEGNACLFCKARRLDDKFYQKLSGQFPDAVFWQELGEILRQLQKQAAEIYNQSLIELYYEIFIKGRGFANASSVEHYLSDVCYTRAAGLFKNAAIASGLRGKVKSNFRLKELKNMKSGLPTTKSDNFPIPLVKQKGGQYTGFEVSSHNDDFIIKIPFGRWQVKKEIDKYRPWEKFDFEQVRKSPRPISLLLSTQRRKRNKGWSKDEGTEAEIRKVMNGDYQTSYIEVKRGSKTGEKSAWMLNLSIDVPKIDKGVDPSIIGGIDVGVKSPLVCAINNAFSRYSISDNDLFRFNKKMFARRRILLKRNRHKRAGHGAKNKLKPISILTGKSERFRKKLIERWACEIADFFIKNKVGTVQMENLESMKRREDSYFNIRLRGFWPYAKMQNKIEFKLKQYGIVVRKVAPNNTSKTCSRCGHPNNYFNFEYRKKNKFPHFKCEKCNFKEDADYNAALNISNPKLKSTKEEP

SEQ ID NO: 872 - protein, 726 aa, synthetic construct
SEVEFSHEYWMRHALTLAKRARDEREVPVGAILVLNNRVIGVGWNRAIGLHDPTAHAEIMALRQGGLVTQNYRLIDATLYVTFEPCVMCAGAMIHSRIGRVVFGVRNSKHGAAGSLVNVLNYPGMNHRVEITEGILADECAALLCDFYRMPRQVFNARKKAQSSINSGGSSGGSSGSETPGTSESPTPESSGGSSGGPAKNTITKTLQLRIVRPYNSAEVEKIVADEKNSREKIALEKNKDKVREACSKHLMVASYCTTQVERNACLFCKARELDGKFYQKLRGQFPDAVFWQELGEIFRQLQKQAAEIYNQSLVELYYEIFVKGKGIANTSRMEHYLSDVCYTRAAKLFKNAAIASGLRGKIKSNFRLKELKSMKSGLPTTRSDNFPIPLVKQKGGQCTGFEISNHDSDFIIKIPFGRWQVKKEIDKYRPWEKFDFEQVRKSPKPISLLLSTQRRKRNKGWSKDEGTEAEIRKVMNGDYQTSYIEVKRGSKIGEKSAWMLNLSIDVPKIDKGVDPSIIGGIDVGVKSPLVCAINNALGRYSISDNDLFHFNKKMFARRRILLKKNRHKRAGHGAKNKLKPITILTEKSKRFRKKLIERWASEIADFFIKNKVGTVQMENLESMKRKEDSYFNIRLRGFWPYAEMQNKIEFKLKQYGIVIRKVAPNNTSKTCSKCGHLNNYFNFEYRKKNKFPHFKCEKCNFKENADYNAALNISNPKLKSTKEEP

SEQ ID NO: 873 - protein, 726 aa, synthetic construct
SEIEFSHEYWMRHALTLAKRARDEREVPVGAVLVLNNRVIGEGWNRAIGLHDPTAHAEIMALRQGGQVMQNYRLTDATLYVTFEPCVMCAGAMIHSRIGRVVFGVRNNKHGAAGSLVNVLNYPGMNHRVEITEGILADECAALLCDFYRMPRQVFNARKKAQSSINSGGSSGGGSGGETPGTSESATQESSGGSSGGSAKNTITKTLKLRIVRPYNSAEVEKIVADEKNNREKIALEMNKDKVKEACSKHLKVAAYCATRVERNACLFCKARKLDDKFYQKLRGQFPDAVFWQEIGEIFRQLQKQAAEIYNQSLIELYYEIFIKGKGFANASSVEHYLSDVCYTRAAELFKNAAVASGLRGKVKSNFRLKELKNMKSGLPTTKSDNFPIPLVKQKGGQYTGFEISSHNDDFIIKIPFGRWQVKKEIDKYRPWEKFDFEQVRKSPKPISLLLSTQRRKRNKGWSKDEGTEAEIRKVMNGDYQTSYIEVKRGSKPGEKSAWMLNLSIDVPKIDKGVDPSIIGGIDVGVKSPLVCAINNAFSRFSISDNDLFRFNKKMFARRRILLKKNRHKRAGHGAKNKLKPISILTGKSERFRKKLIERWACEIADFFIKNKVGTVQMENLESMRRKEDSYFNIRLRGFWPYAEMQNKIEFKLKQYGIEIRKVAPNNTSRTCSKCGHLNNYFNFEYRKKNKFPHFKCEKCNFKEDADYNAALNISNPKLKSTKEEP

SEQ ID NO: 874 - protein, 726 aa, synthetic construct
SEVEFSHEYWMRHALTLAKRARDEREVPVGAVLVLNNRVIGEGWNRAIGLHDPTAHAEIMALRQGGLVMQNYRLTDATLYVTFEPCVMCAGAMIHSRIGRVVFGVRNSKRGAAGSLMNVLNYPCMNHRVEITEGILADECAALLCDFYRMPRQAFNARKKTQSSINPGGSSGGSSGSETPGTSVSATPESSGSSSGGSAKNTITKTLKLRIVRPYNSAEVEKIVADEKNSREKIALEKNKDKVKEACGKHLKVAAYCTTQVERNACLFCKARKLDDKFYQKLRGQFPDAVFWQEIGEIFRQLQKQAAEIYNQSLIELYYEILIKGKGFANASSVEHYLSDVCYTRAAELFKNAAIASGLRGKVKSNFRLKELKNMRSGLPTTKSDNFPIPLVKQKGGQYAGFEISSHNDDFIIKIPFGRWQVKKEIDKYRPWEKFDFEQVRKSPKPISLLLSTRRRKRNKGWSKDEGTEAEIRKVMNGDYQTSYIEVKRGSKTGEKSTWMLNLSIDVPKIDKGVDPSIIGGIDVGVKSPLVCAINNAFSRYSISDNDLFRFNKKMFARRRILLKKNRHKRAGHGAKNKLKPISILTEKSKRFRKKLIERWACEIADFFIKNKVGTVQMENLESMKRKEDSYFNIRLRGFWPYAEMQSKIEFKLKQYGIEIRKVAPNNTSKTCSKCGHLNSYFNFEYRKKNKFPHFKCEKCNFKENADYNAALNISNPKLKSTKEEP

SEQ ID NO: 875 - protein, 726 aa, synthetic construct
SEVEFSHEYWMRHALTLAKRARDEREVPVGAVLVLNNRVIGEGWNRAIGQHDPTAHAEIMALRQGGLVMQNYRLIDATLYVTFEPCVMCAGAMIHSRIGRVVFGVRNSKHGAAGSLMNVLNYPGMNHRVEITEGILADECAALLCDFYHMPRQVFNGRKKAQSSINSGGSSGGSSGSETPGTSESATPESSGGSSSGSTKNTITKTLKLRIVRPYNSTEVEKIVADEKNNREKIALEKNKDKVKEACSRHLKVAAYCTTQVERNACLFCKARKLDDKFYQKLRGQFPDAVFWQEIGEIFRQLQKQAAEIYNQSLIELYYEIFIKGRGFANASSVEHYLSDVCYTRAAELFKNAAIASGLRGKVKSNFRLKELKNMKSGLPTTKSDNFPIPLVKQKGGQYTGFEISSHNDDFIIKIPFGRWQVKKEIDKYRPWEKFDFEQVRKSPKPISLLLSTRRRKRNKGWSKDEGTEAEIRKVMNGDYQTSYIEVKRGSKIGEKSAWMLNLSIDVPKVDKGVDPSIIGGIDVGVKSPLVCAINNAFSRYSISDNELFHFNKKMFARRRILLKKNRHKRAGHGAKNKLKPISVLTEKSGRYRKKLIERWACEIADFFIKNKVGTVQMENLGSMKRKEDSYFNIRLRGFWPYAEMQNKIEFKLKQYGIEIRKVAPDNTSKTCSKCGHLNNYFNFEYRKKNKFPHFKCEKCNFKEDADYNAALNISNPKLKSTKEEP

SEQ ID NO: 876 - protein, 726 aa, synthetic construct
SEVEFGHEYWMRHALTLAKRARDEREVPVGAVLVLNNRVIGVGWNRAIGLHDPTAHAEIMALRQGGLVMQNYRLIDATLYVTFEPCVMCAGAMVHSRIGRVVFGVRNSKRGAAGSLMNVLDYPGMDHRVEITEGILADECAALLCDFYRMPRQVFNARKKAQSSINPGGSSGGSSGSVTPGTSESATPESSGGGFGGSAKNTITKTLQLRIVRPYNSAEVEKIVADEKNNREKIALEKNKDKVKEACSKHLKVASYCTTQVERNACLFCKARKLDDKFYQKLRGQFPDAVFWQELGGIFRQLQKQAAEIYNQSLIELYYEIFIKGKGITNASRVEHYLSDVCYTRAAELFKNAAIASGLRSKVRSNFRLKELKNMKSGLPTTKSDNFPIPLVKQKGGQYTGFEISSHNDDFIIKIPFGRWQVKKEINKYRPWEKFDFEQVRKSPKPISLLLSTQRRKRNKGWSKDEGTEAEIRKVMNGDYQTSYIEVKRGSRIGEKSAWMLSLSIDVPKIDRGVDPGIIGGIDVGVKSPLVCAINNALSRYSISDNDLFHFNKKMFARRRILLKKNRHRRAGHGARNKLKPITVLTEKSKRFRKKLIERWACEVANFFIKNKVGTVQMENLESMKRKEDSYFNIRLRGLWPYAEMQNKIEFKLKQYGIEVRKVAPNNTSKTCSKCGHLNNYFNFEYRKKNKFPPFKCEKCNFKEDADYNAALNISNPKLKGTKEEP

SEQ ID NO: 877 - protein, 726 aa, synthetic construct
SEVEFSHEYWMRHALTLAKRARDEREVPVGAVLVLNNRVIGVGWNRAVGQHDPTAHAEIMALRQGGLVMRNYRLIEATLYVTFEPCIMCAGAMIHSRIGRVVFGVRNSKRGAAGSLMNVLNYPGMNHRVEITEGILADECAALLCDFYRMPRQVLNAQKKAQSSISPGGSSGGSSGSETPGASESVTPKSSGGSSGGSAKNTITKTLKLRIVRPYNSAEVEKIVADEKNHREKIALEKNKGKVKEACSKHLEVAAYCTTQVERNACLFCKARKLDDKFYQKLRGQFPDAVFWQELGEIFRQLQKQAAEIYNQSLIELYYEIFIKGKGFANASSVEHYLSDVCYTRAAELFKNAAIASGLRGKVKSNFRLKELKNMKSGLPTTKSDNFPIPLVKQKGGQYTGFEISSHNDDFIIKIPFGRWQVRKEIDKYRPWEKFDFEQVRKSPKPISLLLSTQRRKRNKGWSKDEGTEAEIRKVMNGDYQTSYIEVKRGSKIGEKGAWMLNLSIDVPKIDKGVDPSIIGGIDVGVKSPLVCAINNALSRYSISDNDLFHFNKKMFARRRILLRKNRHKRAGHGARNKLKPITVLTEKSERFRKKLIERWACEIADFFIKNKVGTVQMENLESMKRKEDSYFNIRLRGFWPYAEMQNKIEFKLKQYGIEIRKVAPNNTSKTCSKCGHLNNYFNFEYRKKNKFPHFKCEKCNFKENADYNAALNISNPKLKGTKEKP

SEQ ID NO: 878 - protein, 726 aa, synthetic construct
SEVEFSHEYWMRHALTLAKRARDEREVPVGAVLVLNNRVIGEGWNRAIGLHDPTAHAEIMALRQGGLVMQNYRLTDAILYATFEPCVMCAGAMIHSRIGRVVFGVRNSKRGAAGSLMNVLNYPGMNHCVKITEGVLVDECAALLCDFYRMPRQVLSAQKKAQSSISSGGSSGGSSGSETPGASESATPKSSVGSSAGSTRNTITKTLKLRIVRPYNSAEVEKIVADEKNNREKIALEKNKDKVKEACSKHLKVAAYCTTQVERNACLFCKARKLDDKFYQKLRGQFPDAVFWQEVGEIFRQLQKQAAEIYNQSLIELYYEIFIKGRGFANASSVEHYLSDVCYTRAAELFKNAAIASGLRGKVKSNFRLKELKNMKSGLPTTKSDNFPIPLVKQKGGQYTGFEISNHNSDFIIKIPFGRWQVKKEINKYRPWEKFDFEQVRKSPKPISLLLSTQRRKRNKGWSKDEGTEAEIRKVMNGDYQTSYIEVKRGSRIGEKSAWMLSLSIDVPKIDRGVDPSIIGGIDVGVKSPLVCAINNTFSRYSISDNDLFHFNKKMFARRRILLKKSKHKRAGHGAKNKLKPITILTEKSGRFRKKLIERWASEIADFFIKNKVGTVQMENLESMKRKEDSYFNIRLRGFWPYAEMQNKIEFKLKQYGIKIRKVAPNNTSKTCSKCGHLNNYFNFEYRKKNKFPHFRCEKCNFKENADYNAALNISNPKLKSTKEEP

SEQ ID NO: 879 - protein, 726 aa, synthetic construct
SEVEFSHEYWMRHALTLAKRARDEREVPVGAVLVLNNRVIGEGWNRAIGLHDPTAHAEIMALRQGGLVMQNYRLSDATLYVTFEPCVMCAGAMIHSRIGRVVFSVRNSKRGAAGSLMNVLNYPGMNHCVEITEGILVDECAALLCDFYRMPRQVLSAQKKAQSSVSSGDSSGGSSGSETPGASGSVTPKSSVGSSAGSTKNTITKTLKLRIVRPYNSAEVEKIVADEKNNREKIALEKNRDKVKEACSKHLKVAAYCTTQVERNACLFCKARKLDDKFYQKLRGQFPDAVFWQELGEILRQLQKQAAETYNQSLIELYYEIFIKGRGFANASSVEHYLSDVCYTRAAELFKNAAIASGLRGKVKSNFRLKELKNMKSGLPTTKSDNFPIPLVKQKGGQYTGFEISSHSDDFIIKIPFGRWQVKKEIDKYRPWEKFDFEQVRKSPKPISLLLSTQRRKRNKGWSKDEGTEAEIRKVMNGDYQTSYIEVKRGSKTGEKSAWMLNLSIDVPKIDKGVDPSIIGGIDVGVKSPLVCAINNAFSRYSISDNDLFRFNKKMFARRRILLKKNRHKRAGHGAKNKLKPISILTGKSERFRKKLIERWACEIADFFIKNKVGTVQMENLESMKRREDSYFNIRLRGFWPYAEMQNKIEFKLKQYGIEIRKVAPINTSKTCSKCGHLNNYFNFEYRKKNKFPHFKCEKCNFKENADYNAALNISNPKLKSTKEEP

SEQ ID NO: 880 - protein, 726 aa, synthetic construct
SEVEFSHEYWMRHALTLARRARDEREVPVGAILVLNNRVIGEGWNRAIGLHDPTAHAEIMALRQGGLVMQNYRLTDATLYVTFEPCVMCAGAMIHSRIGRVVFGVRNSKHGAAGSLVNVLNYPGMNHRVEITEGILADECAALLCDFYRMPRQVFNARKKAQSSINPGGSSGGSSGSETPGTSESATLENSGGSSGGSAKNTITKTLKLRIVRPYNSAEVEKIVADEKNNREKIALEKNKGKVKEACSKHLKMASYCTTQVERNACPFCKARKLDDKFYQKLRSQFPDAVFWQELGEILRQLQKQAAEIYNQSLIELYYEIFIKGRGFANAGSVEHYLSDVCYTRAAELFKNAAIASGLRGKVKSNFRLKELKNMKSGLPTTKSDNFPIPLVKQKGGQYTGFEINSHNDDFIIKIPFGRWQVKKEIDKYRPWEKFDFEQVRKSPKPINLLLSTQRRKRNKGWSKDEGTEAEIRKVMNGDYQTSYIEVKRGSKTGEKSAWMLNLSIDVPKIDKGVDPSIIGGIDVGVKSPLVCAINNAFSRYSISDNDLFRFNKKMFARRRILLKKNRHQRAGHGAKNKLKPITILTEKSGRFRKKLIERWACEIADFFIKNKVGTVQMEDLESMKRREDSYFNIRLRGFWPYAEMQNKIEFKLKQYGIKIRRVAPNNTSKTCSKCGHLNNYFSFEYRKKNKFPHFKCEKCNFKENADYNAALNISNPKLMSTKEEP

SEQ ID NO: 881 - protein, 726 aa, synthetic construct
SEVEFSHEYWMRHALTLAKRARDEREVPVGAVLVLNNRVIGEGWNRAIGLHDPTAHAEIMALRQGGLAMRNYRLVDATLYVTFEPCVLCAGAMVHSRIGRVVFGVRNSKRGAAGSLMNVLNHPGMNHRVEITGGILADECAALLCDFYRMPRQVFNARKKAQSSINPGGSSGGSSGSETPGTSESPTPESSGGSPGGSAKNTITKTLKLRIVRPYNSAEVEKIVADEKNNREKIALEKNKDKVKEACSKHLKVAAYCTTQVERNACLFCKARRLDDKFYQKLRGQFPDAVFWQEIGEIFRQLQKQAAEIYNQSLVELYYEILIKGKGIANASSVEHYLSDVCYTRAAELFKNAAIASGLRNKIKSNFRLKELRNMKSGLPTTKSDNFPIPLVRQKGGQYTGFEISNHNGDFIIKIPFGRWQVKKEINKHRPWEKFDFEQVRKSPKPISLLLSTQRRKRNKGWGKDEGTEAEIRKVMNGDYQTSYIEVKRGSRIGEKSAWMLSLSIDVPKIDRGVDPSIIGGIDVGVKSPLVCAINNALSRYSISDNDLFRFNKKMFARRRILLKKNRHKRAGHGAKNKLKPISILTGKSERFRKKLIERWACEIADFFVKNKVGTVQMENLESMKRREDSYFNIRLRGFWPYAKMLNKIEFKLKQYGVKIRRVAPNNTSKTCSRCGHLNNYFSFEYRKKNKFPHFKCEKCNFKENADYNAALNISNPKLKSTKGEP

SEQ ID NO: 882 - protein, 726 aa, synthetic construct
SEVEFSHEYWMRHALTLARRARDEREVPVGAILVLNNRVIGEGWNRAIGLHDPTAHAEIMALRQGGLVMQNYRLADATLYVTFEPCVMCAGAMIHSRIGRVVFGVRNSKHGAAGSLVNVLNYPGMNHRVEITEGILADECAALLCDFYRMPRQVFNARKKAQSSINPGGSSGGSSGSETPGTSESATLENSGGSSGGSAKNTITKTLKLRIVRPYNSAEVERIVADEKNNREKIALEKNKDKVKEACSKHLKVAAYCTTQVERNACLFCKARRLDDKFYQKLRGQFPDAVFWQEIGEIFRQLQKQAAETYNQSLIELYYEIFIKGKGIANASNVEHYLSDVCYTRAAELFKNAAIASGLRNKIKSNFRLKELRNMKSGLPTTKSDNFPIPLVKQKGGQYTGFEISNHNGDFIIKIPFGRWQAKKEIDKYRPWEKFDFEQVRKSPRPISLLLSTQRRKRNKGWSKDEGTEAEIRKVMNGDYQTSYIEVKRGSKIGEKSAWMLNLSIDVPKIDKGVDPSIIGGIDVGVKSPLVCAINNAFSRYSISDNDLFRFNKKMFARRRILLGKNRHKRAGHGAKNKLKPITILTEKSRRFRKKLIERWASEIADFFIKNKVGTVQMENLESMKRKEDSYFNIRLRGFWPYAEMQNKIEFKLKQYGIEIRKVAPNNTSKTCSKCGHLNNYFNFEYRRKNKFPHFKCEKCNFKENADYNAALNISNPKLKSTKEEP

SEQ ID NO: 883 - protein, 726 aa, synthetic construct
SEVEFSHEYWMRRALTLAKRARDEREVPVGAVLVLNNRVIGVGWNRAIGLHDPTAHAEIMALRQGGLVTQNYRLIDATLYVTFEPCVMCAGAMIHSRIGRVVFGVRNSKHGAAGSLVNVLNYPGMNHRVEITEGILADECAALLCDFYRMPRQVFSARRKAQSSISPGGSSGGSSGGETPGSSKSPTPESPGGSSGGSAKNTITKTLKLRIVRPYNSAEVEKIVADEKNNREKIALEKNKDKVKEACSEHLKVAAYCTTQVERNACLFCKARKLDDKFYLKLRGQFPDAVFWQEIGEIFRQLQKQAAEIYNQSLIELYYEIFIKGKGITNASRVEHYLSDVCYTRAAELFKNAAIASGLRSKVRSNFRLKELKNMKSGLPTTKSDNFPIPLVKQKGGQYTGFEISSHNSDFIIKIPFGRWQVKKEIDKYRPWEKFDFEQVRKSPKPISLLLSTQRRKRNKGWSKDEGTEAEIKKVMNGDYQISYIEVKRGSKIGEKSAWMLNLSVDVPKIDKGVDPSIIGGIDVGVKSPLVCAINNALSRYSISDNDLFHFNKRMFARRRILLRRNRHKRVGHGAKNKLKPISILTEKSERFRKKLIERWACEIADFFIRNKVGTVQMENLEGMKRKEDSYFNIRLRGFWPYAEMQNKIEFKLKQYGIVVRKVAPNNTSKTCSKCGHLNNYFNFEYRKKNKFPHFKCEKCNFKEDADYNAALNISNPKLKSTKGEP

SEQ ID NO: 884 - protein, 726 aa, synthetic construct
SEVEFSHEYWMRHALTLAKRARDEREVPVGAVLVLNNHVIGVGWNRAIGLHDPTAHAEIMALRQGGLVTQNYRLIDATLYVTFEPCIMCAGAMIHSRIGRVVFGVRNSKRGAAGSLMNVLDYPGMNHRVEITEGILADECAALLCDFYRMPRRVFNARKKAQSSINPGGPSGGSSGSETPGTSESPTPESSGGSPGGSAKNTITKTLKLRIVRPYNSAEVEKIVADEKNSREKIALEKNKDKVKEACSKHLKVASYCTTQVERNACLFCKARKLDDKFYQKLRGQFPDAVFWQELGEIFRQLQKQAAEIYNQSLIELYYEIFIKGKGFANASSVEHYLSDVCYTRAAELFKNAAIASGLRGKVKSNFRLKELKNMKSGLPTTKSDNFPIPLVKQKGGQYTGFEISNHNDDFIIKIPFGRWQVKREIDKYRPWEKFDFEQVRKSPKPISLLLSTQRRKRNKGWSKDEGTEAEIRKVMNGDYQTSYIEVKRGSKIGEKSAWMLNLSIDVPKIDKGVDPSIVGGIDVGVKSPLVCAINNAFSRYSIGDNDLFHYNKKMFARRRILLKKNRHKRAGHGAKNKLKPISILTEKSKRFRKKLIERWACEIADFFIKNKVGTVQMENLESMKRKEDSYFNIRLRGFWPYAEMQNKIEFKLKQYGIEVRKVAPNNTSKTCSKCGHLNNYFNFEYRKKNKFPHFKCEKCNFKENADYNAALNISNPKLKSTKEEP

SEQ ID NO: 885 - protein, 726 aa, synthetic construct
SEVEFSHEYWMRHALTLAKRARDEREVPVGAVLVLNNRVIGEGWNRAIGLHDPTAHAEIMALRQGGLVMQNYRLTDATLYVTFEPCVMCAGAMIHSRIGRVVFGVRNSRRGAAGSLMNVLNYPGMNHCVEITEGILVDECAALLCDFYRMPRQVLNAQKKAQSSISSGGSSGGSSGSETPGASESTTPKSSGGSSAGSTKNTITKTLRLRIVRPYNSAEVEKIVADEKNSREKIALERNKDKVKEACSKHLKVASYCTTQVERNACLFCKARKLDDKFYQKLRGQFPDAVFWQELGEIFRQLQKQAAEIYNQSLIELYYEIFIKGKGFANASSVEHYLSDVCYTRAAELFKNAAIASGLRGKVKSNFRLKELKNMKSGLPTTKSDNFPIPLVKQKGGQYTGFEISSHNDDFIIKIPFGRWQVKKEIDKYRPWEKFDFEQVRKSPKPISLLLSTQRRKRNKGWSKDEGTEAEIRRVMNGDYQTSYIEVKRGSKIGEKSAWMLNLSIDVPKIDKGVDPSIVGGVDVGVKSPLVCAINNAFSRYSIGDNDLFHYNKKMFARRRILLKKNRHKRAGHGAKNKLKPITVLTEKSERFRKKLIERWACEIANFFIKNKVGTVQMENLESMKRREDSYFNIRLRGFWPYAEMQSKIEFKLKQYGIKIRKVAPNNTSKTCSKCGHLNNYFNFEFRKKNKFPHFKCEKCNFKEDADYNAALNISNPKLKSTKEEP

SEQ ID NO: 886 - protein, 726 aa, synthetic construct
SGVEFGHEYWMRHALTLARRARDEGEVPVGAVLVLNNRVIGEGWNRAIGLHDPTAHAEIMALRQGGLVMQNYRLVDATLYVTFEPCVLCAGAMVHSRIGRVVFGVRNSKRGAAGSLMNVLNYPGMNHRVEITEGILVDECAALLCDFYRMPRQVLNAQKKAQSSISPDGSSGGSSGSETPGASESVTPKSSGGSSGGSAKNTITKTLKLRIVRPYNSAEVEKIVADEKNNREKIALEKNKGKVKEACSKHLKVAAYCTTQVERNACLFCKARKLDDKFYQKLRGQFPDAVFWQEIGEIFRQLQKQAAEIYNQSLIELYYEIFIKGKGFANASSVEHYLSDVCYTRAAELFKNAAIASGLRGKVKSNFRLKELKNMKSGLPTTKSDNFPIPLVKQKGGQYTGFEISSHNDDFIIKIPFGRWQVKKEIDKYRPWEKFDFEQVRKSPKPISLLLSTQRRKRNKGWSKDEGTEAEIRKVMNGDYQTSYIEVKRGSKIGEKSAWMLSLSIDVPKIDKGVDPSIIGGIDVGVRSPLVCAINNAFSRYSISDNDLFRFNKKMFARRRILLKRNRHKRAGHGAKNKLKPITTLTEKSRRFRKKLIERWACEIADFFIKNKVGTVQMESLESMKRREDSYFNVRLRGFWPYAEMQNKIEFKLKQYGIKIRKVAPNNTSKTCSMCGHLNNYFSFEYRKKYKFPHFKCEKCNFKENADYNAALNISNPKLMSTKEGP

SEQ ID NO: 887 - protein, 726 aa, synthetic construct
SEVEFSHEYWMRHALTLAKRARDEREVPVGAILVLNNRVIGEGWNRAIGLHDPTAHAEIMALRQGGLVMQNYRLIDATLYVTFEPCVMCAGAMVHSRIGRVVFGVRNSKRGAAGSLMNVLDYPGMGHRVEITEGILADECAALLCDFYCMPRQVFNAQKRAQSSINSGGSSGGSSGSETPGTSESATPGSSGGGSSSSAKNTITKTLQLRIVRPYNSAEVEKIVADEKDNREKIALEKNKDKVKEACSKHLKVASYCTTQVERNACPFCKARKLDDKFYQKLRGQFPDAVFWQELGEIFRQLQKQAAEIYNQSLIELYYEIFIKGKGFANASSVEHYLSDVCYTRAAELFKNAAIASGLRGKVKSNFRLKELKNMRSGLPTTKSDNFPIPLVKQKGGQYTGFEISSHNGDFIIKIPFGRWQVKKEINKHRPWERFDFEQVRKSPKPISLLLSTQRRKRNKGWSKDEGTEAEIRKVMNGDYQTSYIEVKRGSKIGEKSAWMLNLSIDVPKIDKGVDPCIIGGIDVGVKSPLVCAINNAFSRYSISDNDLFRFNKKVFARRRILLKKNRHKRAGHGTKNKLKPITILTEKSGRFRKKLIERWACEIANFFVKNKVGTVQMEDLESMKRKEDSYFNIRLRGFWPYAEMQNKIEFKLKQYGIEIRKVAPNNTSKTCSKCGHLNNYFNFEYRKKNKFPHFKCEKCNFKENADYNAALNICNPKLKSTKEEP

SEQ ID NO: 888 - protein, 726 aa, synthetic construct
SEVEFSHEYWMRHALTLAKRARDEREVPVGAVLVLNNRVIGEGWNRAIGLHDPTAHAEIMALRQGGLVMQNYRLTDATLYVTFEPCVMCAGAMIHSRIGRVVFGVRNSKRGAAGSLMNVLNYPGMNHCVEISEGILADECAALLCDFYRMPRQVFNARKKAQSSINPGGSSGGSSGSETPGTSESATPESSGGSSGSSAKNTITKTLKLRIVRPYNSAEVEKIVADEKNNREKIALEKNKDKVKEACSKHLKVAAYCTTQVERNACLFCKARRLDDKFYQKLRGQFPDAVFWQEIGEIFRQLQKQAAEIYNQSLIELYYEIFIKGKGIANASSVEHYLSDVCYTRAAELFKNAAIASGLRNKVKSNFRLKELRSMKSGLPTTKSDNFPIPLVRQKGGQYTGFEISNHNSDFIIKIPFGRWQAKKEIDKYRPWEKFDFEQVRKSPKPISLLLSTQRRKRNKGWSKDEGTEAEIKKVMNGDYQTSYIEVKRGSKIGEKSAWMLSLSIDVPKIDKGVDPSIIGGIDVGVKSPLVCAINNAFGRHSISDNDLFHFNKKMFARRRILLKKNRHKRAGHGAKNKLKPITVLTEKSVRFRKKLIERWACEIADFFIKNKVGTVQMENLESMKRKEDSYFNIRLRGFWPYAEMQNKIEFKLKQYGIEIRKVAPNNTSKTCSKCGHLNNYFSFEYRKKNKFPHFKCEKCNFKENADYNAALNISNPKLKSTKEEP

SEQ ID NO: 889 - protein, 726 aa, synthetic construct
SEVEFSHEYWMRHALTLAKRARDEREVPVGAVLVLNNRVIGEGWNRAIGLHDPTAHAEIMALRQGGLVLQNYRLVDATLYVTFEPCVMCAGAMIHSRIGRVVFGVRNSKHGAAGSLMNVLNYPGMNHRVEITEGILADECAALLCDFYRMPHQVFSARKKAQSSISPGGSSGGSSGSETPGTSESATPESSGGSSGGSAKNTITKTLKLRIVRPYNSAEVEKIVADEKNNREKIALEKNKDKVKEACSKHLKVAAYCTTQVERNACLFCKARKLDDKFYQKLRGQFPDAVFWQEIGEIFRQLQKQAAEIYNQSLIELYYEIFIKGKGFANASSVEHYLSDVCYTRAAELFKNAAIASGLRGKVKSNFRLKELKNMRSGLPTTKSDNFPIPLVKQKGGQYTGFEISSHNDDFIIKIPFGRWQVKEEIDKYRPWEKFDFEQVRKNPKPISLLLSIQRRKRNKGWSRDEGTEAEIRKVMNGDYQTSYIEVKRGSKIGEKSAWMLNLSIDVPKIDKGVDPSIIGGIDVGVKSPLVCAINNAFSRYSISDNDLFHFNKKMFARRRILLKKNRHKRAGHGAKNKLWPITILTEKSKRFRKKLIERWACEIADFFIKNKVGTVQMENLEGMKRKEDSYFNIRLRGFWPYAEMQNKIEFKLKQYGIEIRKVAPNNTSKTCSKCGHLNNYFDFEYRKKNKFPHFKCEKCNFKENADYNAALNISNPKLKSTKEGP

SEQ ID NO: 890 - protein, 726 aa, synthetic construct
SEVEFSHEYWMRHALTLAKRARDEREVPVGAVLVLNNRVIGEGWNRAIGLHDPTAHAEIMALRQGGLAMQNYRLVDATLYVTFEPCVLCAGAMVHSRIGRVVFGVRNSKRGAAGSLMNVLNHPGMNHRVEITGGILADECAALLCDFYRMPRQVFNAQKKARSNINSGGSSGGSSGSETLGTSESVTPESSGGSSGGSAKNTITKTLKLRIVRPYNSAEVEKIVADEKNNREKIALEKNKDKVKEACSEHLKVAAYCTTQVERNACLFCKARKLDDKFYQKLRGQFPDAVFWQEISEIFRQLQKQAAEIYNQSLIELYYEIFIKGKGFANASSVEHYLSDVCYTRAAELFKNAAIASGLRGKVKSNFRLKELKSMKSGLPTTKSDNFPIPLVKQKGGQYTGFEISNHNSDFIIKIPFGRWQAKKEIDKYRPWEKFDFEQVRKSPKPISLLLSTQRRKRNRGWSKDEGTEAEIKKVMNGDYQTSYIEVKRGSKVGEKSAWMLNLSIDVPKIDKGVDPSIIGGIDVGVKSPLVCAINNAFSRYSISDNDLFRFNKKMFARRRILLKKNRHKRAGHGAKNKLKPITILTGKSRRFRKKLIERWACEIADFFIKNKVGTVQMESLESMKRKEDSYFNIRLRGFWPYAEMQNKIEFKLKQYGIKIRKVAPNNTSKTCSRCGHLNNYFNFEYRRKNKFPHFKCEKCNFKENADYNAALNISNPKLKSTKEEP

SEQ ID NO: 891 - protein, 726 aa, synthetic construct
SEVEFSHEYWMRHALTLAKRARDEREVPVGAVLVLNNRVIGEGWNRAIGLHDPTAHAEIMALRQGGLVIQNYRLSDATLYVTFEPCVMCAGAMIHSRIGRVVFGARNSKRGAAGSLMNVLNYPGMNHCVEITEGILVDECAALLCDFYRMPRQVLSAQKKAQSSISSGGSSGGSSGSETPGASGSVTPKSSVGSSAGSTKNTITKTLKLRIVRPYNSAEVEKIVVDEKNNREKVALEKNKDKVKEACSEHLKVAAYCTTQVERSACLFCKARKLDDKFYQKLRGQFPDAVFWQEIGEIFRQLQKQAAEIYNQSLIELYYEIFIKGKGFANASSVEHHLSDVCYTRAAELFKNAAIASGLRGKVKSNFRLKELKNMKSGLPTTKSDNFPIPLVKQKGGQYTGFEISSHNGDFIIKIPFGRWQAKKEIDKYRPWEKFDFEQVRKSPKPISLLLSTQRRKRNKGWSKDEGTEAEIRKVMNGDYQTSYIEVKRGSKIGEKSAWMLNLSIDVPKIDKGVDPGIIGGIDVGVKSPLVCAINNASSRYSISDNDLFHFNKKMFARRRILLKKNRHKRAGHGAKNKLKPITIMTEKSKRFRKKLIERWACELADFFIKNKVGTVQMENLESMKRKEDSYFNIRLRGFWPYAEMQNKIEFKLKQYGIEIRKVAPNNTSKTCSKCGHLNNYFNFEYRKKNKFPHFKCEKCNFKEDADYNAALNISNPKLKSTKEEP

SEQ ID NO: 892 - protein, 726 aa, synthetic construct
SEVEFSHEYWMRHALTLAKRARDEREVPVGAILVLNNRVIGEGWNRAIGLHDPTAHAEIMALRQGGLVMQNYRLIDATLYVTFEPCVMCAGAMIHSRIGRVVFGVRNSKHGAAGSLVNVLNYPGMNHRVEITEGILADECAALLCDFYRMPRQVFNARKKAQSSINPSGSSGGSSGSVTPGTSESATPESSGGGFGGSAKNTITKTLKLRIVRPYNSAEVEKIVADEKNSREKIALEKNKDKVKEACSEHLKVAAYCTTQVERNACLFCKARKLDDRFYQKLRGQFPDAVFWQEIGEIFRQLQKQAAEIYNQSLIELYYEIFIKGKGFANASSVEHYLSDVCYTRAAELFKNAAIASGLRGKVKSNFRLKELRNMKSGLPTTKSDNFPIPLVRQKGGQYTGFEISNHNGDFIIKIPFGRWQVKKEICKHRPWEKFDFEQVRKSPKPISLLLSTQRRKRNKGWSKDEGTEAEIRKVMNGDYQTSYIEVKRGSKIGEKSAWMLNLSIDVPKIDKGVDPSIIGGIDVGVKSPLVCAINNALSRYSISDNDLFHFNKKMFARRRILLRKNRHKRAGHGARNKLKPITVLTEKSERFRKKLIERWACEIANFFIKNKVGTVQMENLESMKRREDSYFNIRLRGFWPYAEMQSKIEFKLKQYGIKIRKVAPNNTSKTCSKCGHLNNYFNFEFRKKNKFPHFKCEKCNFKEDADYNAALNISNPKLKGTKEEP

SEQ ID NO: 893 - protein, 726 aa, synthetic construct
SEVEFSHEYWMRHALTLAKRARDEREVPVGAVLVLNNRVIGVGWNRAIGLHDPTAHAEIMALRQGGLVMQNYRLIDATLYVTFEPCIMCAGAMIHSRIGRVVFGVRNSKRGAAGSLMNVLNYPGMNHRVEITEGVLADECAALLCDFYRMPRQVLNAQKKAQSSINSGGSSGGGSGGETPGTSESATQESSGGSSGGSAKNTITKTLKLRIVRPYNNAEVEKIVADEKNNREKIALEKSKDKVKEACSKHLKVAAYCTTQVERNACLFCKARKLDDKFYQKLRGQFPDAVFWQEIGEIFRQLQKQAAEVYNQSLVELYYEILIKGKGIANASSVEHYLSDVCYTRAAELFKNAAIASGLRNKIKSNFRLKELRNMKSGLPTTKSDNFPIPLVRQKGGQYTGFEISNHDGDFIIKIPFGRWQVKKEINKHRPWEKFDFEQVRKSPKPISLLLSTQRRKRNKGWSKDEGTEAEIRKVMNGDYQTSYIEVKRGSKIGEKSAWMLNLSIDVPKIDKGVDPSIIGGIDVGVKSPLVCAINNALSRYSISDNDLFHFNKKMFARRRILLRKNRHKRAGHGAKNKLKPITIMTEKSKRFRKKLIERWACEIADFFIKNKVGTVQMENLESMKRREDSYFNIRLRGFWPYAEMQNKIEFKLKQYGIVVRKVAPNNTSKTCSKCGHLNNYFSFEYRKKNKFPHFKCEKCNFKENADYNAALNISNPKLKSTKEEP

SEQ ID NO: 894 - protein, 726 aa, synthetic construct
SEVEFSHEYWMRHALTLAKRARDEREVPVGAVLVLNNRVIGEGWNRAIGLQDPTAHAEIMALRQGGLVMQNYRLSDATLYVTFEPCVMCAGAMIHSRIGRVVFGVRNSKRGAAGSLMNVLNYPGMNHCVEITEGILVDECAALLCDFYRMPRQVLSAQRKAQSSVSSGGSSGGSSGSETPGASGSVTPKSSVGSSAGSTKNTITKTLKLRIVRPYNSAEVEKIVADEKNNREKIALEKNKDKVKEACSRHLKVASYCTTQVERNACLFCKARKLDDKFYQKLRGQFPDAVFWQELGEIFRQLQKQAAEIYNQSLIELYYEIFIKGKGFANASSVEHYLSDVCYTRAAELFKNAAIASGLRGKVKSNFRLKELKNMKSGLPTTKSDNFPIPLVKQKGGQYTGFEISSHNDDFIIKIPFGRWQVRKEIDKYRPWEKFNFEQVRKSPKPISLLLSTQRRKRNKGWSKDEGTEAEIRKVMNGDYQTSYIEVKRGSKIGEKSAWMLSLSIDVPKIDKGVDPSIIGGIDVGVKSPLVCAINNAFNRYSISDNNLFHFNKKMFARRRILLKKNGHKRAGHGAKNKLKPITILTEKSKRFRKKLIERWACEIADFFIKNKVGTVQMENLESMKRKEDSYFNIRLRGFWPYAEMQNKIEFKLKQYGIEIRKVAPNNTSKTCSKCGHLNNYFNFEYRRKNKFPHFKCEKCNFKEDADYNAALNISNPKLKSTKGEP

SEQ ID NO: 895 - protein, 726 aa, synthetic construct
SEVEFSHEYWMRHALTLAKRARDEREVPVGAVLVLNNRVIGEGWNRAIGLHDPTAHAEIMALRQGGLVMQNHRLIDATLYVTFEPCVLCAGAMVHSRIGRVVFGVRNSKRGAAGSLMNVLNCPGMNHRVEITEGVLADECAALLCDFYRMPRQVFNAQKKAQSSINSGGSSGGNSGSETPGASESVTPKSSGGSSGGSAKNTITKTLKLRIVRPYNSAEVEKIVADEKNNREKIALEKNKGKVKEACSKHLEVAAYCTTQVERNACLFCKARKLDDKFYQKLRGQFPDAVFWQELGEIFRQLQKQAAEIYNQSLIELYYEIFIKGKGFANASSVEHYLSDVCYTRAAELFKNAAIASGLRGKVKSNFRLKELKNMKSGLPTTKSDNFPIPLVKQKGGQYTGFEVSSHNDDFIIKIPFGRWQEKKEINKYRPWEKFDFEQVRKSPKPISLLLSTQRRKRNKGWSKDEGTEAEIKKVMNGDYQTSYIEVKRGSKIGEKSAWMLNLSIDVPKIDKGVDPSIIGGIDVGVKSPLVCAINNAFSRYSISDNDLFHFNKKMFARRRILLKKGKHKRAGHGAKNKLKPITILTEKSGRFRKKLIERWACEIADFFIKNKVGTVQMENLESMKRKEDSYFNIRLRGFWPYAEMQNKIEFKLKQYGIGIRKVAPNNTSKTCSKCGHLNNYFNFEYRKKNKFPHFKCEKCNFKENADYNAALNISNPKLKSTKEEP

SEQ ID NO: 896 - protein, 726 aa, synthetic construct
SEVEFSHEYWMRHALTLAKRARDEREVPVGAILVLNNRVIGEGWNRAIGLHDPTAHAEIMALRQGGLVMQSYRLADATLYVTFEPCVMCAGAMIHSRIGRVVFGVRNSKHGAAGSLMNVLNYPGMNHRVEITEGILADECAALLCDFYRMPRRVFNAQKRAQSSINSGGSSGGSSDSETPGTSESATPESSGGGSSGSAKDTITKTLQLRIVRPYNSAEVEKIVADEKNNREKIALEKNKDKVKEACSKHLKVAAYCTTQVERNACPFCKARKLDDKFYQKLRGQFPDAVFWQELGGIFRQLQKQAAEIYNQSLIELYYEIFIKGRGFANASSVEHYLSDVCYTRAAELFKNAAIASGLRGKVKSNFRLKELKNMKSGLPTTKSDNFPIPLVKQKGGQYTGFEISSHNDDFIIKIPFGRWQVKKEIDKYRPWEKFDFEQVRKSPKPISLLLSTQRRKRNKGWSKDEGTEAEIRKVMNGDYQTSYIEVKRGSKTGEKSAWMLNLSIDVPKIDKGVDPSIVGGIDVGVKSPLVCAINNAFSRYSISDNDLFRFNKKVFARRRILLKKNRHRRAGHGAKNKLKPITILTEKSKRFRKKLIERWACEIADFFIKNKVGIVQMENLESMKRREDSYFNIRLRGFWPYAEMQNKIEFKLKQYGIEVRKVAPNNTSKTCSKCGHLNYYFNFEYRKKNKFPHFKCEKCNFKEDADYNAALNISSPKLKSTKEEP

SEQ ID NO: 897 - protein, 726 aa, synthetic construct
SEVEFSHEYWMRHALTLAKRARDEREVPVGAVLVLNNRVIGEGWNRTIGLHDPTAHAEIMALRQGGLVMQNYRLTDATLYVTFEPCVMCAGAMIHSRIGRVVFGVRNSKRGAAGSLMNVLNYPGMNHCVEITEGILVDECAALLCDFYRMPRQVLNAQKKAQSSISSGGSSGGSSGSETPGASESVTPKSSVGSSAGSTKNTITKTLKLRIVRPYNSAEVEKIVADEKNNRERIALEKNKDKVKEACSKHLKVAAYCTTQVERNACLFCKARRLDDKFYQKLRGQFPDAVFWQEIGEIFRQLQKQAAEIYNQSLVELYYEIFIKGKGIANASSVEHYLSDVCYTRAAELFRNAAIASGLRNKIKSNFRLKELRNMKSGLPTTKSDNFPIPLVRQKGGQYTGFEISNHNGDFIVKIPFGGWQVKKEISKHRPWEKFDFEQVRKSPKPISLLLSTQRRKRNKGWGKDEGTEAEIRKVMNGDYQTSYIEVKRGSKIGEKSAWMLNLSIDVPKIDKGVDPSIIGGIDVGVKSPLVCAINNALSRYSISDNDLFHFNKKMFARRRILLRKNRHKRAGHGAKNKLKPITIMTEKSKRFRKKLIERWACEIADFFIKNKVGTVQMENLESMKKKEDSYFNIRLRGFWPYAEMQNKIEFKLKQYGIVVRKVAPNNTSKTCSKCGHLNNYFNFEYRKKNKFPHFKCEKCNFKEDADYNAALNISNPKLKSTRGEP

SEQ ID NO: 898 - protein, 726 aa, synthetic construct
SEVEFSHEYWMRHALTLAKRARDECEVPVGAVLVLNNRVIGEGWNRAIGLHDPTAHAEIMALRQGGLVMQNHRLVDATLYVTFEPCVLCAGAMVHSRIGRVVFGVRNSKRGAAGSLMNVLNYPGMNHRVEITEGILADECAALLCDFYRMPRQVFNAQKKARSNTNSGDSSGGSSGSGIPGTSESATPESSGGSSGGSAKNTITKTLKLRIVRPYNSAEVEKIVADEKNNRERIALEKNKDKVKEACSKHLKVAAYCTTQVERNACLFCKARRLDDKFYQKLRGQFPDAVFWQEIGEIFRQLQKQAAEIYNQSLIELYYEIFIKGKGFANASSVEHYLSDVCYTRAAELFKNAAIASGLRGKVKSNFRLKELKNMKSGLPTTKSDNFPIPLVKQKGGQYTGFEISSHNDDLIIKIPFGRWQVKKEIDRYRPWEKFDFEQVRKSPKPISLLLSTQRRKRNKGWSKDEGTEAEIRKVMNGDYQTSYIEVKRGSKIGEKSAWMLNLSIDVPKIDKGVDPSIIGGIDVGVKSPLVCAINNAFSRYSISDNDLFHFNKKMFARRRILLKKNRHKRAGHGAKNKLKPISILTEKSKRFRKKLIERWACEIADFFIKNKVGTVQMENLESMKRKEDSYFNIRLRGFWPYAEMQNKIEFKLKQYGIEIRKVAPNNTSRTCSKCGHLNNYFNFEYRRKYKFPHFKCEKCNFKEDADYNAALNISNPKLKSTKEEP

SEQ ID NO: 899 - protein, 726 aa, synthetic construct
SEVEFSHEYWMRHALTLAKRARDEREVPVGAVLVLNNRVIGEGWNRAIGLHDPTAHAEIMALRQGGLVLQNYRLIDATLYVTFEPCVMCAGAMIHSRIGRVVFGVRNNKHGAAGSLVNVLNYPGMNHRVEITEGILANECAALLCDFYRMPRQVFNARKKAQSSINPGGSSGGSSGSETPGTSESATPESTGGSSGGSAKNTITKTLKLRIVRPYNSAEVEKIVADEKNNREKIALEKNKDKVKEACSKHLKVASYCTTQVERNACPFCKARKLDDKFYQKLRGQFPEAVFWQEIGEIFRQLQKQAAEIYNQSLIELYYEIFIKGKGFANASSVEHYLSDVCYTRAAELFKNAAIASGLRGKVKSNFRLKELKNMKSGLPTTKSDNFPIPLVRQKGGQYTGFEISSHNDDFIIKIPFGRWQVKKEIDKYRPWEKFDFEQVRKSPKPISLLLSTQRRKRNKGWSKDEGTEAEIRKVMNGDYQTSYIEVKRGSRIGEKSAWMLSLSIDVPKIDRGVDPSIIGGIDVGVKSPLVCAINNALSRYSISDNDLFHFNKKMFARRRILLKKTRHKRAGHGTKNKLKPISILTEKSERFRKKLIERWACEIADFFIKNKVGTVQMENLEGMKRKEDSYFNIRLRGFWPYAEMQNKIEFKLKQYGIEIRKVAPNNTSKTCSKCGHLNNYFNFEYRKKNKFPHFKCEKCNFKENADYNAALNISNPKLKSTKEEP

SEQ ID NO: 900 - protein, 726 aa, synthetic construct
SEVEFSHEYWMRHALTLAKRARDEREVPVGAVLVLNNRVIGEGWNRAIGLHDPTAHAEIMALRQGGLVMQNYRLIDATLYVTFEPCVMCAGAMIHSRIGRVVFGVRNSKRGAAGSLMNVLNYPGMNHCVEITEGILMDECAALLCDFYRMPRQVLSAQKKAQSSISSGGPSGGSSCSETPGASGSPTPESSGGSSGGSAKNTITKTLKLRIVRPYNSAEVEKIVADEKNNREKIALEKNKDKVKEACSEHLKVATYCTTQVERNACLFCKARKLDDKFYQKLRGQFPDAVFWQEIGEIFRQLQKQAAEIYNQSLIELYYEIFIKGKGFANASSVEHYLSDVCYTRAAELFKNAAIASGLRGKVKSNFRLKELKNMKSGLPTTKSDNFPIPLVKQKGGQYTGFEISSHNDDFIIKIPFGRWQMKKEVDKYRPWEKFDFEQVRKSPKPISLLLSTQRRKRRKGWSKDEGTEAEIRKVMNGDYQTSYVEVKRGSKIGEKSAWMLNLSIDVPKIDKGVDPSIVGGIDVGVKSPLVCAIDNALSRYSISDNDLFHFNKKMFARRRILLKKNRHKRAGHGAKNKLKPISILTGKSERFRKKLIERWACEIADFFIKNKVGTVQMENLESMKRKEDSYFNIRLRGFWPYAEMQNKIEFKLKQYGIEIRKVAPSNTSKTCSKCGHLNNYFNFEYRKKNKFPHFKCEKCNFKENADYNAALNISNPELKSTKEEP

SEQ ID NO: 901 - protein, 726 aa, synthetic construct
SEVEFSHEYWMRHALTLAKRARDEREVPVGAVLVLNNRVIGEGWNRAIGLHDPTAHAEIMALRQGGLVMQNYRLSDATLYVTFEPCVMCAGAMIHSRIGRVVFGVRNSKRGAAGSLMNVLNYPGMNHCVEITEGILVDECAALLCDFYRMPRQVLSAQKKAQSSISSGGSSGGSSGSETPGASGSVTPKSSVGSSAGSTKNTITKTLKLRIVRPYNSAEVEKIVADEKNNREKIALEKNRDKVKEACSKHLKVAAYCTTRVERNACLFCKARKLDDKFYQKLRGQFPDAVFWQELGGIFRQLQKQAAEIYNQSLIELYYEIFIKGRGFANASSVEHYLSDVCYTRAAELFKNAAIASGLRGKVKSNFRLKELKNMKSGLPTTKSDNFPIPLVKQKGGQYTGFEISSHNDDFIIKIPFGRWQVKKEIDKYRPWEKFDFEQVRRSPKPISLLLSTQRRKRNKGWSKDEGTEAEIRKVMNGDYQTSYIEVKRGSKTGEKSAWMLNLSIDVPKIDRGVDPSIIGGIDVGVKSPLVCAINNAFGRYSISDNDLFRFNKKMFARRRILLKKSRHKRAGHGAKNKLKPISILTERSKRFRKKLIERWACEIADFFIKNKVGTVQMENLESMKRKEDSYFNIRLRGLWPYAEMQNKIEFKLKQYGIEIRKVAPNNTSKTCSKCGHLNNYFNFEYRKKNKFPHFKCEKCNFKENADYNAALNISNPKLKSTKGEP

SEQ ID NO: 902 - protein, 726 aa, synthetic construct
SEVEFSHEYWMRHALTLAKRARDEREVPVGAVLVLNNRVIGVGWNRAIGLHDPTAHAEIMALRQGGLVMQNYRLTDATLYVTFEPCVMCAGAMIHSRIGRVVFGVRNSKRGAAGSLMNVLNYPGMNHCVEITEGILVDECAALLCDFYRMPRQVLNAQKKAQSSISSGGSSGGSSGSETPGASGSVTPKSSGGSSAGSTKDTITKTLQLRIVRPYNSAEVEKIVADEKNNREKIALEKNKDKVKEACGKHLKVASYCTTQVERNACLFCRARKLDDKFYQKLRGQFPDAVFWQEIGEIFRQLQKQAAEIYNQSLIELYYEIFIKGKGFANASSVEHYLSDVCYTRAAELFKNAAIASGLRGKVKSNFRLKELKNMKSGLPTTKSDNFPIPLVKQKGGQYTGFEISNHNSDFIIKIPFGRWQVKKEINKYRPWEKFDFEQVRKSPKPISLLLSTQRRKRNKGWSKDEGTEAEIRKVMNGDYQTSYIEVKRGSKTGEKSAWMLNLSIDVPKIDKGVDPSIIGGIDVGVKSPLVCAINNAFNRYSISDNNLFHFNKKMFARRRILLKKNRHKRAGHGAKNKLKPISILTEKSERFRKKLIERWACEIADFFIRNKVGTVQMENLEGMKRREDSYFNIRLRGFWPYAEMQNKIEFKLKQYGIEVRKVAPNNTSKTCSKCGHLNNYFSFEYRKKNKFPHFKCEKCNFKENADYNAALNISNPKLKSTKEEP

SEQ ID NO: 903 - protein, 726 aa, synthetic construct
SEVEFSHEYWMRHALTLAKRARDEREVPVGAVLVLNNRVIGEGWNRTTGLHDPTAHAEIMALRQGGLVMRNYRLTDATLYVTFEPCVMCAGAMIHSRIGRVVFGVRNSKRGAAGSLMNVLDYPGMNHCVEITEGILVDECAALLCDFYRMPRQVLNARKKAQSSISSGGSSGGCSGSEMPGASESVTPKSSGGSSAGSTKNTITKTLKLRIVRPYNSAEVEKIVADEKNSREKIALERNKDKVKEACSEHLKVAAYCTTQVERNACLFCKARKLDDRFYQKLRGQFPDAVFWQETGEIFRQLQRQAAEIYNQSLIELYYEIFIKGKGFANASSVEHYLSDVCYTRAAELFKNAAIASGLRGKVKSNFRLKELKNMKSGLPTTKSDNFPIPLVKQKGGQYTGFEISSHNDDFIIKIPFGRWQVKKEIDKYRPWEKFDFEQVRKSPKPISLLLSTQRRKRNKGWSKDEGTEAEIRKVMNGDYQTSYIEVKRGSKTGEKSAWMLNLSIDVPKIDKGVDPSIIGGIDVGVKSPLVCAINNAFSRYSISDNDLFRFNKKMFARRRILLKKNRHKRAGHGAKNKLKPISILTGKSERFRKKLIERWACEIADFFVKNKVGTVQMENLESMKRKEDSYFNIRLRGFWPYAEMQNRIEFKLKQYGIKVRKVAPNNTSKTCSKCGHLNNYFNFEYRKKNKFPYFKCEKCNFKENADYNAALNISNPKLKSTKEEP

SEQ ID NO: 904 - protein, 726 aa, synthetic construct
SEVEFSHEYWMRHALTLAKRARDEREVPVGAVLVLNNRVIGGGWNRTVGLHDPTAHAEIMALRQGGLVMQNCRLVDATLYVTFEPCVMCAGAMIHSRIGRVVFGVRNSKRGAAGSLMNVLNYPGTNHRVEITEGILADECAALLCDFYRMPRRVFNAQKKARSNISPGGSSGGSGGSETPGASESATPKSSVGSSAGSTKNTITKTLKLRIVRPYNSAEVEKIVADEKNNREKIALEKNKDKVKEACSKHLKMASYCTTQVERNACLFCKARKLDDKFYQKLRGQFPDAVFWQELGGIFRQLQKQAAEIYNQSLIELYYEIFIKGRGFANASSVEHYLSDVCYTRAAELFKNAAIASGLRGKVKGNFRLKELKNMKSGLPTTKSDNFPIPLVKQKGGQYTGFEISSHNDDFIIKIPFGRWQVKKEIDKYRPWEKFDFEQVRKSPKPISLLLSTQRRKRNKGWSRDEGTEAEIRKVMNGDYQTSYIEVKRGSKTGEKSAWMLNLSIDVPKINKGVDPSIIGGIDVGVKSPLVCAINNAFSRYSISDNDLFRFNKKVFARRRILLKKNRHRRAGHGAKNKLKPITILTEKSKRFRKKLIERWACEIADFFIKNKVGTVQMENLESMKRKEDSYFNIRLRGFWPYAEMQNKIEFKLKQYGIEIRKVAPNNTSRTCSKCGHLNNYFSFEYRRKNKFPHFKCEKCNFKEDADYNAALNISNPKLKSTKEEL

SEQ ID NO: 905 - protein, 726 aa, synthetic construct
SEVEFSHEYWMRHALTLAKRARDEREVPVGAVLVLNNRVIGEGWNRAIGLHDPTAHAEIMALRQGGLAMQNYRLVDATLYVTFEPCVLCAGAMVHSRIGRVVFGVRNSRRGAAGSLMNVLNHPGMNHRVEITGGILADECAALLCDFYRMPRQVFNAQKKARSNINSGGSPGGSSGSVTPGTSESATPESSGGGFGGSAKNTITKTLQLRIVRPYNSAEVEKIVTDEKDNREKIALEKNKDKVKEACSKHLKMASYCTTQVERNACLFCKARELDVKFYQKLRGQFPDAVFWQELGGILRQLQKQAAEIYNQSLIELYYEIFIKGKGIANASRVEHYLSDVCYTRAAELFKNAAIASGLRSKVRSNFRLKELKNMKSGLPTTKSDNFPIPLVKQKGGQYTGFEISSHNSDFIIKIPFGRWQVKEEIDKYRPWEKFDFEQVRKSPKPISLLLSTQRRQKNKGWSKDEGTEAEIRRVMNGDYQTSYIEVKRGSKIGEKSTWMLNLSIDVPKIDKGVDPSIIGGIDVGVKSPLVCAINNAFGRYSISDNDLFHFNKKMFARRRILLKKNRHKRAGHGAKNKLKPISILTEKSKRFRKKLIERWACEIADFFIKNKVGTVQMENLESMKRKEDSYFNIRLRGFWPYAEMQNKIEFKLKQYGIEIRKVAPNNTSKTCSKCGHLNSYFNFEYRKKNKFPHFKCEKCNFKENADYNAALNISNPKLKSTKEEP

SEQ ID NO: 906 - protein, 726 aa, synthetic construct
SEVEFSHEYWMRHALTLAKRARDEREVPVGAVLVLNNRVIGEGWNRTTGLHDPTAHAEIMALRQGGLVMRNYRLTDATLYVTFEPCVMCAGAMIHSRIGRVVFGVRNSKRGAAGSLMNVLNYPGMNHCVEVTEGILVDECAALLCDFYRMPRQVLNAQKKAQSSISPGGSSGGSSGSETPGASESVTPKSSGGSSGGSAKNTITKTLKLRIVRPYNSAEVEKIVADEKNNREKIALEKNKDKVKEACSKHLKVASYCTTQVERNACLFCKARKLDDKFYQKLRGQFPDAVFWQELGEIFRQLQKQAAEIYNQSLVELYYEIFVKGKGFANASSVEHYLSDVCYTRAAELFKNAAIASGLRGKVKSNFRLKELKNMKSGLPTTKSDNFPIPLVKQKGGKYTGFEISSHNDDFIIKIPFGRWQVKKEIDKYRPWEKFDFEQVRKSPKPISLLLSTQRRKRNKGWSKDEGTEAEIRKVMNGDYQTSYIEVKRGSKIGEKSAWMLNLSIDVPKIDKGVDPSIIGGIDVGVKSPLVCAINNAFSRYSISDNDLFHFNKKMFARRRILLKKNRHKRAGHGAKNKLKPISILTEKSKRFRKKLIERWACEIADFFIKNKVGTVQMENLEGMKRKEDSYFNIRLRGFWPYAEMQNKIEFKLKQYGIVIRKVAPNNTSKTCSRCGHLNNYFNFEYRKKNKFPHFKCEKCNFKENADYNAALNISNPKLKSTKEEP

SEQ ID NO: 907 - protein, 726 aa, synthetic construct
SEDEFSHEYWMRHALTLAKRARDGREVPVGAVLVLNNRVIGEGWNRAIGLHDPTAHAEIMALRQGGLVMQNYRLTDATLYVTFEPCVMCAGAMIHSRIGRVVFGVRNSKRGAAGSLMNVLNYPGMNHCVEITEGILVDECAALLCDFYRMPRQVLNAQKKAQPSISSGGSTGGSSGSETPGASESVTPKSSGGSSIGSTKNTITKTLKLRIVRPYNSAEVEKIVADEKNSREKIALEKNKDKVKEACSEHLKVAAYCTTQVERNACLFCKARKLDDRFYQKLRGQFPDAVFWQELGEIFRQLQKQAAEIYNQSLIELYYEIFIKGKGFANASNVEHYLSDVCYTRAAELFKNAAIASGLRGKVKSNFRLKELKNMKSGLPTTKSDNFPIPLVKQKGGQYTGFEISSHNDDFIIKIPFGRWQVRKEIDKYRPWEKFDFEQVRKSPKPINLLLSTQRRKRNKGWSKDEGTEAEIKKVMSGDYQTSYIEVKRGSKAGEKSAWMLSLSIDVPKIDKGVDPCTIGGIDVGVKSPLVCAINNAFSRYSVSDNDLFHFNKKMFARRRILLKKNRHKRAGHGAKNKLKPISILTEKSKRFRKKLIERWACEIADFFIKNKVGTVQMENLESMKRKEDSYFNIRLRGFWPYAEMQNKIEFKLKQYGIVVRKVAPNNTSKTCSQCGHLNNYFDFEYRKKNKFPYFKCEKCNFKENADYNAALNISNPQLKSTKGEP

SEQ ID NO: 908 - protein, 726 aa, synthetic construct
SEVEFSHEYWMRHALILAKRARDEREVPVGAVLVLNNRVIGEGWNRAIGLHDPTAHAEIMALRQGGLVMQNYRLIDATLYVTFEPCVMCAGAMIHSRIGRVVFGVRNNKHGAAGSLVNVLNYPGMNHRVEITEGILADECAALLCDFYRMPRQVFNARKKAQSSINPGGSSGGSSGSETPGTSESATPESSGGSSGGSAKNTITKTLKLRIVRPYNSAEVEKIVADEKNSREKIALEKNKDKVKEACSRHLEVAAYCTTQVERNACLFCKARKLDDKFYQKLRGQFPDAVFWQEIGEIFRQLQKQAAEIYNRSLIELYYEIFVKGKGFANASSVEHYLSDVCYTRAAELFKNAAIASGLRGKVKSNFRLRELKSMRSGLPTTKSDNFPIPLVKQKGGQYTGFEISSHNDDFIIKIPFGRWQVKKEIDKYRPWEKFDFEQVRKSPKPISLLLSTQRRKRNKGWSKDEGTEAEIRKVMNGDYQTSYIEVKRGSKIGEKSAWMLSLSIDVPKIDKGVNPSIIGGIDVGVKSPLVCAINNAFSRYSISDNDLFHFNKKMFARRRILLKKNRHKRAGHGAKNKLKPLTILTGKSKRFRKKLIERWACEIADFFIKNKVGTVQMENLESMKRREDSYFNIRLRGFWPYAEMQNKIEFKLKQYGIEIRKVAPNNTSKTCSKCGHLNNYFNFEYRKKNKFPHFKCEKCNFKENADYNAALNISNPKLKSTKEKP

SEQ ID NO: 909 - protein, 726 aa, synthetic construct
SEVEFSHEYWMRHALTLAKRARDEREVPVGAILVLNNRVIGEGWNRAIGLHDPTAHAEIMALRQGGLVTQNYRLIDATLYVTFEPCVMCAGAMIHSRVGRVVFGVRNSKHGAAGSLMNVLNYPGMNHRVEITEGILADECAALLCDFYRMPRRVFNARKKAQSSIDPGGPFGGSSGSGTPGTSESATPESSGGSSGGSAKNTITKTLKLRIVRPYNSTEVEKIVADEKNNREKIALEKNKDKVREACSKHLKVASYCTTQVERNACLFCKARKLDDKFYQKLRGQFPDAVFWQELGEIFRQLQKQAAEIYNQSLIELYYEIFIKGRGFANASSVEHYLSDVCYTRAAELFKNAAIASGLRGKVKGNFRLKELKNMKSGLPTTKSDNFPIPLVKQKGGQYTGFGISNHNGDFIIKIPFGRWQVKKEIDKYRPWEKFDFEQVRKSPKPISLLLSTQRRKRNRGWGKDEGTEAEIKRVMNGDYQTSYIEVKRGSKIGEKSAWMLNLSIDVPKIDKGVDPRIIGGIDVGVKSPLVCAINNAFSRYSISDNDLFHFNKKMFARRRILLKKNRHKRAGHGTKNKLKPISILTEKSKRFRKKLIERWACEIADFFIKNKVGTVQMENLESMKRKEDSYFNIRLRGFWPYAEMQNKIEFKLKQYGIEIRKVAPNNTSKTCSKCGHLNNYFSFEYRRKNKFPHFKCEKCNFKEDADYNAALNISNPKLKSTKEEP

SEQ ID NO: 910 - protein, 726 aa, synthetic construct
SEVEFSHEYWMRHALTLAKRARDEREVPVGAILVLNNRVIGEGWNRAIGLHDPTAHAEIMALRQGGLVMQNYRLIDATLYVTFEPCVMCAGAMIHSRIGRVVFGVHNSKHGAAGSLVNVLNYPGMNHRVEITEGILADECAALLCDFYRMPRQVFNARKKAQSSINPSGSSGGSSGSVTPGTSESATPESSGGGSSGSARNTITKTLQLRIVRPYNSAEVEKIVADEKNNREKIALEKYKDKVKEACSEHLKVAAYCTTQVERNACLFCKARKLDDRFYQKLRGQFPGAVFWQEIGEIFRQLQKQAAEIYNQSLIELYYEIFIKGKGFANASSVEHYLSDVCYTRAAELFKNAAIASGLRGKVKSNFRLKELKNMKSGLPTTKSDNFPIPLVKQKGGQYTGFEISNHNSDFIIKIPFGRWQAKKEIDKYRPWEKFDFEQVRKSPKPISLLLSTQRRKRNKGWSKDEGTEAEIRKVMNGDYQTSYIEVKRGSKTGEKSAWMLNLSIDVPKIDKGVDPSIIGGIDVGVKSPLVCAINNAFSRYSISDNDLFRFNKKMFARRRILLKKNRHKRAGHGAKNKLKPITILTEKSKRFRKKLIERWACEIADFFIKNKVGTVQMESLESMKRKEDSYFNIRLRGFWPYAEMQNKIEFKLKQYGIEIRKVAPNNTSKTCSKCGHLNNYFNFEYRKKNKFPHFKCEKCSFVENADYNAALNISNPKLKSTKEEP

SEQ ID NO: 911 - protein, 726 aa, synthetic construct
SEVGFSHEYWMRHALTLAKRARDEREVPVGAVLVLNNRVIGEGWNRAIGQHDPTAHAEIMALRQGGLVMQNYRLTDATLYVTFEPCVMCAGAMIHSRIGRVVFGVRNSKHGAAGSLVNVLNYPGMNHHVEITEGILADECAALLCDFYRMPRQVFNARKKAQSSINPGSSSGGSSGSETPGASGSVTPKSSGGSSAGSTKDTITKTLKLRIVRPYNSAEVEKIVADEKNSREKIALEKNKDKVKEACSKHLEVAAYCTTQVERNACLFCKARKLDDKFYQKLRGQFPDAVFWQELGEIFRQLQKQAAEIYNQSLIELYYEIFIKGKGFANASSVEHYLSDVCYTRAAELFKNAAIASGLRGKVKSNFRLKELKNMKSGLPTTKSDNFPIPLVKQKGGQYTGFEISSHNDDFIIKIPFGRWQVKKEIDKYRPWEKLDFEQVRKSPKPISLLLSTQRRKRNKGWSKDEGTEAEIRKVMNGDYQTSYIEVKRGSKIGEKSAWMLNLSIDVPKIDKGVDPSIVGGIDVGVRSPLVCAIDNVLSRYSISDNDLFHFNKKMFARRRILLKKNRHRRAGHGAKNKLKPITVLTEKSERFRKKLIERWACEIANFFIKNKVGTVQMENLESMKRREDSYFNIRLRGFWPYAEMQSKIEFKLKQYGIKIRKVAPNNTSKTCSKCGHLNNYFNFEFRKKNKFPHFKCEKCNFKEDADYNAALNISNPKLKGTKEEP

SEQ ID NO: 912 - protein, 726 aa, synthetic construct
SEVEFSHEYWMRHALTLAKRARDEREVPVGAVLVLNNRVIGEGWNRTTGLHDPTAHAEIMALRQGGLVMQNHRLVDATLYVTFEPCVMCAGAMIHSRIGRVVFGVRNSKRGAAGSLTNVLNYPGMNHRVEITEGILVDECAALLCDFYRMPRQVFNAQKKAQSTINSGGSSGGSSGSETPGTSESPTPESSGGSPGGSAKNTITKTLKLRIVRPYNSAEVEKIVAEEKNNREKIALEKNKDKVKEACSKHLKVAAYCTTQVERNACPFCKARKLDDKFYQKLRGQFPDAVFWQELGEILRQLQKQAAEIYNQSLIELYYEIFIKGRGFANASSVEHYLSDVCYTRAAELFKNAAIASGLRGKVKSNFRLKELKNMKSGLPTTKSDNFPIPLVKQKGGQYTGFEISSHNDDFIIKIPFGRWQVKKEIDKYRPWEKLDFEQVRKSPKPISLLLSTQRRKRNKGWSKDEGTEAEIRKVMNGDYQTSYIEVKRGSKIGEKSAWMLNLSIDVPKIDKGVDPSIIGGIDVGVKSPLVCAINNALSRYSISDNDLFHFNKKMFARRRILLRKNRHKRAGHGAKNKLKPITIMTEKSKRFRKKLIERWACEIADFFIKNKVGTVQMENLESMKRKEDSYFNIRLRGFWPYAEMQNRIEFKLKQYGIEIRKVAPNNTSKTCSKCGHLNNYFNFEYRRKNKFPHFKCEKCNFKENADYNAALNICNPRLKGTKEEP

SEQ ID NO: 913 - protein, 726 aa, synthetic construct
SEDEFSHEYWMRHALTLAKRARDGHEVPVGAVLVLNNRVIGEGWNRAIGLHDPTAHAEIMALRQGGLVMQNYRLIDATLYVTFEPCVMCAGAMVHSRIGRVVFGVRNSKRGAAGSLMNVLDYPGMGHRVEITEGILADECAALLCDFYCMPRQVFNAQKRTQSSINSGGSSGGSSGSETPGTSESATPESSGGGPSGSAKNTITKTLQLRIVRPYNSAEVEKIVADEKNNREKIALEKNKDKVKEACSKHLKVASYCTTQVERNACPFCKARKLDDKFYQKLRGRFPDAVFWQELGEILRQLQKQAAEIYNQSLIELYYEIFIKGRGFANASSVEHYLSDVCYTRAAELFKNAAIASGLRGKVKSNFRLKELKNMKSGLPTTKSDNFPIPLVKQKGGQYTGFEISSHDDDFIIKIPFGRWQVKKEIDKYRPWEKFDFEQVRKSPKPISLLLSTQRRRRNKGWSKDEGTEAEIRKMMNGDYQTSYIEVKRGSKTGEKSAWMLNLSIDVPKIDKGVDPSIIGGVDVGVKSPLVCAINNAFSRYSISDNDLFRFNKKMFARRRILLKKNRHKRAGHGAKNKLKPISILTGKSERFRKKLIERWACEIADFFIKNKVGTVQMENLESMKRKEDSYFNIRLRGFWPYAEMQNKIEFKLKQYGIEVRKVAPNNTSKTCSKCGHLNNYFNFEYRKKNKFPHFKCEKCNFKENADYNAALNISNPKLKSTKEEP

SEQ ID NO: 914 - protein, 726 aa, synthetic construct
SEVEFSHEYWMRHALTLAKRARDEREVPVGAVLVLNNRVIGVGWNRAIGLHDPTAHAEIMALRQGGLVMQNYRLIDATLYVTFEPCVMCAGAMIHSRIGRVVFGVRNSKHGAAGSLVNVLNYPGMNHRVEITEGILADECAALLCDFYRMPRQVFGARRKAQSSINPGGSSGGSSVSETPGTSESPTPESPGGSSGGSAKNTITKTLKLRIVRPYNSAEVEKIVADEKNNREKIALEKNKDKVKEACSKHLKVAAYCTTQVERNACLFCKARRLDDKFYQKLRGQFPDAVFWQEIGEIFRQLQKQAAEIYNQSLVELYYEILIKGKGIANAGSVEHYLSDVCYTRAAELFKNAAIASGLRNKIKSNFRLKELKNMKSGLPTTKSDNFPIPLVKQKGGQYTGFEISNHNGDFIIKVPFGRWQARKEIDKYRPWEKFDFEQVRKSPKPISLLLSTQRRKRNRGWGKDEGTEAEIKKVMNGDYQTSYIEVKRGSKIGEKSAWMLNLSIDVPKIDKGVDPSIIGGIDVGVKSPLVCAINNAFGRYSISDNDLFHFNKKMFARRRILLKKNRHKRAGHGAKNKLKPITILSEKSKRFRKKLIERWACEIADFFIKNKVGTVQMENLESMKRKEDSYFNIRLRGFWPYAEMQDKIEFKLKQYGIVIRKVAPNSTSKTCSRCGHLNNYFNFEYRRKNKFPHFKCEKCNFKENADYNAALNISNPKLKSTKEEP

SEQ ID NO: 915 - protein, 726 aa, synthetic construct
SEVEFSHEYWMRHALTLAKRARDEREVPVGAVLVLNNRVIGEGWNRAIGLHDPTAHAEIMALRQGGLVMQNYRLIDATLYVTFEPCVMCAGAMIHSRIGRVVFGVRNNKHGAAGSLVNVLNYPGMNHRVEITEGILADECAALLCDFYRMPRQVFNARKKAQSSINPGGPSGGSSGSETPGTSESATPESSGGSSAGSIKDTITKTLKLRIVRPYNSAEVEKIVADEKNSREKIALEKNKDKVKEACSEHLKVAAYCTTQVERNACLFCKARKLDDRFYQKLRGQFPDAVFWQEIGEIFRQLQKQAAEIYNQSLIELYYEIFIKGKGFANASSVEHYLSGVCYTRAAELFKNAAIASGLRGKVKSNFRLKELKNMKSGLPTTKSDNFPIPLVKQKGGQYTGFEISNHNSDFIIKIPFGRWQAKKEIDKYRPWEKFDFEQVRKSPKPISLLLSTQRRKKNRGWSKDEGTEAEIKKVMNGDYQTSYIEVKRGSKIGEKSAWMLSLSIDVPKIDKGVDPSIIGGIDVGVKSPLVCAISNAFSRYSISDNDLFHFNKKMFARRRILLKKSKHKRAGHGAKNKLKPITILTEKSRRFRKKLIERWACEIADFFIKNKVGTVQMENLESMKRKEDSYFNIRLRGFWPYAEMQSKIEFKLKQYGIEIRRVAPNNTSRTCSKCGHLNNYFNFEYRKKNKFPHFKCEKCNFKEDADYNAALNISNPKLKSTKEEP

SEQ ID NO: 916 - protein, 726 aa, synthetic construct
SEVEFSHEYWMRHALTLAKRARDGREVPVGAVLVLNNRVIGEGWNRAIGLHDPTAHAEIMALRQGGLVMQNYRLIDATLYVTFEPCAMCAGAMVHSRIGRVVFGVRNSKRGAAGSLMNVLNYPGMDHRVEITEGILVDECAALLCDFYRMPRQVLNAQKKAQSSISSGGSSGGCSGSEMPGASESVTPKSSGGSSAGSTKNTITKTLKLRIVRPYNSAEVEKIVADEKNSREKIALERNKDKVKEACSEHLKVAAYCTTQVERSACLFCKARKLDDKFYQKLRGQFPDAVFWQELGEIFRQLQKQAAEIYNQSLIELYYEIFIKGKGFANASSVEHYLSDVCYTRAAELFKNAAIASGLRGKVKSNFRLKELKNMKSGLPTTKSDNFPIPLVKQKGGQYTGFEISSHNDDFIIKIPFGRWQVKKEIDKYRPWEKFDFEQVRKSPKPISLLLSTQRRKRNKGWSKDEGTEAEIRKVMNGDYQTSYIEVKRGNKTGEKSAWMLNLSIDVPKIDKGVDPSIIGGIDVGVKSPLVCAINNAFSRYSISDNDLFHFNKKMFARRRILLKKNRHKRAGHGAKNKLKPISILTEKSKRFRKKLIERWACEIADFFIKNKVGTVQMENLESMKRKEDSYFNIRLRGFWPYAEMQNKIEFKLKQYGIEIRKVAPNNTSKTCSKCGHLNNYFNFEYRKKNKFPHFKCEKCYFKEDADYNAALNISNPKLRSTKEEP

SEQ ID NO: 917 - protein, 726 aa, synthetic construct
SEVEFSHEYWMRHALTLAKRARDEREVPVGAILVLNNRVIGEGWNRAIGLHDPTAHAEIMALRQGGLVMQNYRLIDATLYVTFEPCVMCAGAMIHSRIGRVVFGVRNSKHGAAGSLVNVLNYPGMNHRVEITEGILADECAALLCDFYRMPRQVFNAQKRAQSSINSGGSSGGSSGSDTPGTSESATPESSGGGSSGSAKNTITKTLQLRIVRPYNSAEVEKIVADEKNNREKIALEKNKDKVREACSKHLKVAAYCTTQVERNACLFCKARRLDDKFYQKLRGQFPDAVFWQEIGEIFRQLQKQAAEIYNQSLVELYYEIFIKGKGIANASSVEHYLSDVCYTRAAELFKNAAIASGLRNKIKSNFRLKELRNMKSGLPTTKSDNFPIPLVRQKGGQYTGFEISNHNGDFIIKIPFGRWQVKKEISKHRPWEKFDFEQVRKSPKPISLLLSTQRRKRNKGWGKDEGTEAEIRKVMNGDYQTSYIEVKRGSKIGEKSAWVLNLSIDVPKIDKGVDPSIIGGIDVGVKSPLVCAINNAFSRYSISDNDLFHFNKKMFARRRILLKKNGHKRAGHGAKNKLKPVTILTEKSGRFRKKLIERWACEIADFFIKNKVGTVQMENLESMRRREDSYFNIRLRGFWPYAEMQNKIEFKLKQYGIKIRKVAPNNTSKTCSKCGHLNGYFNFEYRKRNKFPRFKCEKCNFKEDADYNAALNISNPKLKSTKEEP

SEQ ID NO: 918 - protein, 726 aa, synthetic construct
SEVEFSHEYWMRHALTLAKRARDEREVPVGAVLVLNNRVIGEGWNRAIGLHDPTAHAEIMALRQGGLVLQNYRLVDATLYVTFEPCVLCAGAMVHSRIGRVVFGARNSKRGAAGSLMNILNYPGMNHRVEITEGILADECAALLCDFYRMPRQVFNAQKKAQSSINSGGSSGGSSGSETPSTSESATPESSGGSSGGSAKNTITKTLQLRIVRPYNSAEVEKIVTDEKNNREKIALEKNKDKVKEACSKHLKMASYCTTQVERNACLFCKARKLDDKFYQKLRGQFPDAVFWQELGGIFRQLQKQAAEIYNQSLIELYYEIFIKGKGITNASRVEHYLSDVCYTRAAELFKNAAIASGLRSKVRSNFRLKELKNMKSGLPTTKSDNFPIPLVKQKGGQYTGFEISSHNSDFIIKIPFGRWQVKEEIDKFRPWEKFDFEQVRKSPKPISLLLSTQRRKKNKGWSKDEGTEAEIRRVMSGDYQTSYIEVKRGSKIGEKSAWMLNLSIDVPKIDKGVDPSIIGGIDVGVKSPLVCAINNSSSRYSISDNDLFRFNKKMFARRRILLRKNRHKRAGHGAKNKLKPISILTGKSERFRKKLIERWACEIADFFIKNKVGTVQMENLESMKRKEDSYFNIRLRGFWPYAEMQNKIEFKLKQYGIEIRKVAPNNTSKTCSKCGHLNNYFNFEYRKKNKFPHFKCEKCNFKENADYNAALNISNPKLKSTTEEP

SEQ ID NO: 919 - protein, 726 aa, synthetic construct
SEVEFSHEYWMRHALTLAKRARDEREVPVGAILVLNNRVIGEGWNRAIGLHDPTAHAEIMALRQGGLVMQNYRLIDATLYVTFEPCVMCAGAMIHSRIGRVVFGVRNNKHGAAGSLVNVLNYPGMNHRVEITEGILADECAALLCDFYRMPRQVFNARKKAQSSINPGGSSGGSSGSETPGTSESATPESSGGGSGGSAKNTITKTLKLRIVRPYNSAEVEKIVADEKNNREKIALEKNKDKVKEACSKHLKVASYCTTQVERNACPFCKARKLDDKFYQKLRGQFPDAVFWQELGEILRQLQKQAAEIYNQSLIELYYEIFIKGRGFANASSVEHYLSDVCYTRAAELFKNAAIASGLRGKVKSNFRLRELKNMKSGLPTTKSDNFPIPLVKQKGGQYTGFEISSHNDDFIIKIPFGRWQVKKEIDKYRPWEKFDFEQVRKSPKPISLLLSTQRRKRNKGWSKDEGTEAEIRKVMNGDYQTSYIEVKRGSKIGEKSAWMLNLSIDVPKIDKGVDPSIIGGIDVGVKSPLVCAINNAFSRYSISDNDLFRFNKKAFARRRILLKKNGHKRAGHGTKNKLKPITIMTEKSKRFRKKLIERWACEIADFFIKNKVGTVQMENLESMKRKEDSYFNIRLRGFWPYAELQNKIEFKLKQYGIVVRKVAPNNTSKTCSKCGHLNNYFNFEYRKKNKFPHFKCEKCNFKENADYNAALNISNPKLKSTKEGP

SEQ ID NO: 920 - protein, 726 aa, synthetic construct
SEVEFSHEYWMRHALTLAKRARDEREVPVGAVLVLNNRVIGEGWNRAIGLHDPTAHAEMMALRQGGLVMQNYRLIDATLYVTFEPCVMCAGAMIHSRIGRVVFGVRNSKHGAAGSLVNVLNCPGMNHRVEITEGILADECAALLCDFYRMPRQVFNARKKAQSSISSGGSSGGSSGSETPGASESVTPKSSGGSSAGSTKNTITKTLKLRIVRPYNSAEVEKIVADEKNNREKIALERNRDKVKEACSKHLKVASYCTTQVERNACLFCKARKLDDKFYQKLRGQFPDAVFWQELGEIFRQLQKQAAEIYNQSLIELYYEIFIKGKGLANASSVEHYLSDVCYTRAAELFKNAAIASGLRGKVKSNFKLKELKSMKSGLPSTKSDNFPIPLVKQRGGQYTGFEISSHNDDFIIKIPFGRWQAKKEIDKYRPWEKFDFEQVRKSPKPISLLLSTQRRKRNRGWSKDEGTEAEIRKVMNGDYQTSYIEVKRGSKIGEKSAWMLNLSIDVPKIDKGVDPSIIGGIDVGVKSPLVCAINNAFSRYSISDNDLFRFNKKMFARRRILLGKNRHKRAGHGVKNKLKPITILTEKSGRFRKKLIERWACEIADFFVKNKVGTVQMENLESMKRKEDSYFNIRLRGFWPYAEMQNKIEFKLKQYGIVVRKVAPNNTSKTCSKCGHLNNYFNFEYRKKNKFPHFKCEKCNFKEDADYNAALNISNPKLKSTKGEP

SEQ ID NO: 921 - protein, 726 aa, synthetic construct
SEVEFSHEYWMRHALTLAKRARDEREVPVGAVLVLNNRVIGEGWNRAIGLHDPTAHAEIMALRQGGLVMQNYRLTDATLYVTFEPCVMCAGAMIHSRIGRVVFGVRNSKRGAAGSLMNVLNYPGMNHCVEITEGILVDECAALLCDFYRMPRQVLTAQKKAQSSINPGGSSGGSSGSETPGTGESAIPESSGGSSGGSARNTITKTLKLRIVRPYNSAEVEKIVADEKNNREKIALEKNKDKVKEACSKHLKVAAYCTTQVERSACLFCKARRLDDKFYQKLRGQFPDAVFWQETGEIFRQLQRQAAEIYNQSLIELYYEIFIKGKGFANASSVEHYLSDVCYTRAAELFKNAAIASGLRGKVKSNFRLKELKNMKSGLPTTKSDNFPIPLVKQKGGQYTGFEISSHNDDFIIKIPFGRWQVRKEIDKYRPWEKFDFEQVRKSPKPISLLLSTQRRKRNKGWSKDEGTEAEIRKVMNGDYQTSYIEVKRGSKIGEKSAWMLSLSIDVPKIDKGVDPRIIGGIDVGVRSPLVCAINNAFSRYSISDNDLFRFNKKMFARRRILLKKNRHKRAGHGAKNKLKPITILTEKSRRFRKKLIERWACEIANFFVKNKVGTVQMENLESMKRKEDSYFNIRLRGFWPYAEMQNKIEFKLKQYGIKIRKVAPNNTSKTCSKCGHLNNYFSFEYRKKNKFPHFKCEKCNFKEDADYNAALNISNPKLKSTKEEP

SEQ ID NO: 922 - protein, 726 aa, synthetic construct
SEVEFSHEYWMRHALTLAKRARDEREVPVGAVLVLDNRVIGEGWNRAIGLHDPTAHAEIMALRQGGLVMQNYRLSDATLYVTFEPCVMCAGAMIHSRISRVVFGVRNSKRGAAGSLMNVLNYPGMNHCVKITEGILVDECAALLCDFYRMPRQVLSAQKKAQSSVSSGGSSGGSSGSETPSASGSVTPKSSVGSSAGSTKNTITKTLQLRIVRPYNSAEVEKIVADEKNNREKIALEKNKDKVKEACSKHLKVAAYCTTQVERNACLFCKARRLDDKFYQKLRGQFPDAVFWQEIGEIFRQLQKQAAEIYNQSLIELYYEIFIKGKGFANASSVEHYLSDVCYTRAAELFKNAAIASGLRGKVKSNFRLKELKNMKSGLPTTKSDNFPIPLVKQKGGQYTGFEISSHNDDFIIKIPFGRWQVRKEIDKYRPWEKYNFEQVRKSPKPISLLLSTQRRKRNRGWSKDESTEAEIKKVMNGDYQTSYIEVKRGSKIGEKSAWMLNLSIDVPKIDKGVDPSIIGGIDVGVKSPLVCAVNNAFSRYSISDNDLFHFNKKVFARRRILLKKNRHRRAGHGAKNKLKPITILTEKSKRFRKKLIERWACEIADFFIKNKVGTVQMENLESMKRKEDSYFNIRLRGFWPYAEMQNKIEFKLKQYGIKIRKVAPNNTSRICSKCGHLNNYFSFEYRKKNKFPHFKCEKCNFKEDADYNAALNISNPKLKGTKGEL

SEQ ID NO: 923 - protein, 726 aa, synthetic construct
SEVEFSHEYWMRHALTLAKRARDEREVPVGAVLVLNNRVIGEGWNRAIGLHDPTAHAEIMALRQGGLVMQNYRLTDATLYVTFEPCVMCAGAMIHSRIGRVVFGVRNSKRGAAGSLMNVLNYPGMNHCVEITEGILMDECAALLCDFYRMPRQVLNAQKKAQSSISSGGSSGGSSGSKTPGASGSVTPKSSGGSSAGSTKDTITKTLKLRIVRPYNSAEVEKIVADEKNSREKIALEKNKDKVKEACSEHLKVAAYCTTQVERNACLFCKARKLDDGFYQKLRGQFPDAVFWQEIGEIFRQLQKQAAEIYNQSLIELYYEIFIKGKGFANASSVEHYLSDVCYTRAAELFKNAAIASGLRGKVKSNFRLKELKNMKSGLPTTKSDNFPIPLVKQKGGQYAGFEISSHNDDFVIKIPFGRWQVKKEIDKYRPWEKFDFEQVRKSPKPISLLLSTQRRKRNKGWSKDEGTEAEIKKVMNGDYQTSYIEVKRGSKIGEKGAWMLNLSIDVPKIDKGVDPSIIGGIDVGVKSPLVCAINNAFSRYSISDNDLFRFNKKMFARRRILLKKNSHKRAGHGARNKLKPITILTEKSERFRKKLIERWASEIADFFIKNKVGTVQMENLESIKRREDNYFNIRLRGFWPYAEMQNKIEFKLKQYGIEVRKVAPNNTSKTCSKCGHLNNYFNFEYRKKNKFPLFKCEKCNFKENADYNAALNISNPKLKSTKEEP

SEQ ID NO: 924 - protein, 726 aa, synthetic construct
SEVEYSHEYWMRYALTLAKRARDEREVPVGAVLVLNNRVIGEGWNRAIGLHDPTAHAEIMALRQGGLVMQNYRLIDATLYVTFEPCVMCAGAMIHSRIGRVVFGVRNSKRGAAGSLMNVLNYPGMNHRVEITEGILADECAALLCDFYRMPRQVLNAQKRARSCINSGGSSGGSSGSETPGTSESATPETPGGSSGGSAKNTITKTLKLRIVRPYNSAEVEKIVADEKDNRERIALEKNKGKVKEACSKHLKVAAYCTTQVERNACLFCKARKLDDKFYQELRGQFPDAVFWQGIGEIFRQLQKQAAEIYNQSLIELYYEIFIKGKGITNASRVEHYLSDVCYTRAAELFKNAAIASGLRSKVRSNFRLKELKNMKSGLPTTKSDNFPIPLVKQKGGQYTGFEISSHNDDFIIKIPFGRWQVKKEIDKYRPWEKFDFEQVRKSPKPISLLLSTQRRKRNKGWSKDEGTEAEIRKVMNGDYQTSYIEVKRGSKTGEKSAWMLNLSIDVPKIDKGVDPSIIGGIDVGVKSPLVCAINNALSRYSVSDNDLFRFNKKMFARRRILLKKNRHKRAGHGAKNKLKPITILTKKSERFRKKLIERWACEIADFFIKNKVGTVQMENLESMKRKEDSYFNIRLRGFWPYAEMQNKIEFKLKQYGIEIRKVAPNNTSKTCSKCGHLNNYFNFEYRKKNKFPHFKCEKCNFKEDADYNAALNISNPKLKSTRGEP

SEQ ID NO: 925 - protein, 725 aa, synthetic construct
SEDEFSHEYWMRHALTLAKRARDGREVPVGAVLVLNNRVIGEGWNRAIGLHDPTAHAEIMALRQGGLVMQNYRLTDATLYVTFEPCVMCAGAMIHSRIGRVVFGVRNSKRGAAGSLMNVLNYPGMNHCVEITEGILSGECAALLCDFYRMPRQVFNAQKKAQSNINSGGSSGGSSGNETPGTSESPTPESSGGSSGGSAKNTITKTLKLRIVRPYNSTEVEKIVADEKNNREKIALEKNKGKVKEACSEHLKVAAYCTTQVERNACLFCKARKLDDRFYQKLRGQFPDAVFWQEIGEIFRQLQKQAAEIYNQSLIELYYEIFIKGKGFANASSVEHYLSDVCYTRAAELFKNAAIASGLRGKVKSNFRLRELKNMKSGLPTTKSDNFPIPLVKQKGGQYTGFEISNHNSDFIIKIPFGRWQVKKEINKYRPWEKFDFEQVRKSPKPISLLLSTQRRRRNKGWSKDEGTEAEIRKVMNGDYQISYIEVKRGSRIGEKSAWMLSLSIDVPKIDRGVDPSIIGGIDVGVKSPLVCAINNALSRYSISDNDLFHYNKKMFARRRILLKKNRLKRAGHGAKNKLKPISILTEKSKRFRKKLIERWACEIADFFIKNRVGTVQMENLESMKRKEDSYFNIRLRGFWPYAEMQNKIEFKLKQYGIVVRKVAPNNTSKTCSKCGHLNNYFNFEYRKKNKFPHFKCEKCNFREDADYNAALNISNPKLSTKGEP

SEQ ID NO: 926 - protein, 726 aa, synthetic construct
SEVEFSHEYWMRHALTLAKRARDEREVPVGAILVLNNRVIGEGWNRAIGLHDPTAHAEIIALRQGGLVMQNYRLIDATLYVTFEPCVMCAGAMIHSRIGRVVFGVRNSKHGAAGSLVNVLNYPGMNHHVGITEGILADECAALLCDFYRMPRQVFSARKKAQSSINPGGSSGGSSGSETPGTSESATPESSGGSSGGSARNTITKTLKLRIVRPYNSAEVEKIVADEKNNREKIALEKNKDKVKEACSKHLKVAAYCTTQVERNACLFCKARKLDDKFYQKLRGQFPDAVFWQELGGIFRQLQKQAAEVYNQSLVELYYEILIKGKGIANASSVEHYLSDVCYTRAAELFKNAAIASGLRNKIKSNFRLKELRNMKSGLPTTKSDNFPIPLVRQKGGQYTGFEISNHDGDFIIKIPFGRWQVKKEINKHRPWEKFDFEQVRRSPKPISLLLSTQRRKRNKGWSKDEGTEAEIRKVMNGDYQTSYIEVKRGSKIGEKGAWMLNLSIDVPKIDKGVDPSIIGGIDVGVKSPLVCAINNAFSRYSISDNDLFRFNKKMFARRRILLGKNRHKRAGHGVKNKLKPITILTEKSGRFRKKLIERWACEIADFFVKNKVGTVQMENLESMKRKEDSYFNIRLRGFWPYAEMQNKIEFKLKQYGIKVRKVAPNNTSKTCSKCGHLNNYFSFEYRKKNKFPHFKCEKCNFKENADYNAALNISNPKLKSTKEEP

SEQ ID NO: 927 - protein, 726 aa, synthetic construct
SEVEFSHEYWMRRALTLAKRARDEREVPVGAVLVLNNRVIGVGWNRAVGLHDPTAHAEIMALRQGGLVMQNYRLIEATLYVTFEPCIMCAGAMIHSRIGRVVFGVRNSKRGAAGSLMNVLNYPGMNHRVEITEGILADECAALLCDYYRMPRQVFNARKKAQSSINSGGSPGGSSDSETPGASESVTPKSSVGGSAGSTKNTITKTLKLRIVRPYNSAEVEKIVADEKDNREKIALERNKDKVKEACSKHLKVAAYCTTQVERNACLFCKARKLDDEFYQKLGGQFPDAVFWQELGEILRQLQKQAAEIYNQSLIELYYEIFIKGRGFANASSVEHYLSDVCYTRAAELFKNAAIASGLRGKVKSNFRLKELKNMKSGLPTTKSDNFPIPLVKQKGGQYTGFEISSHNDDFIIKIPFGRWQVKKEIDKYRPWEKFDFEQVRKSPKPISLLLSTQRRKRNRGWSKDEGTEAEIKKVMNGDYQTSYIEVKRGSKTGEKSAWMLNLSIDVPKIDKGVDPSIIGGIDVGVKSPLVCAINNALSRYSISDNDLFHYNKKMFARRRILLKKNRHKRAGHGAKNKLRPISILTEKSKRFRKKLIERWACEIADFFIKNKVGTVQMENLESMKRKEDSYFNIRLRGFWPYAEMQNKIEFKLKQYGIEIRKVAPNNTSKTCSKCGHLNSYFDFEYRKKNKFPHFKCEKCNFKENADYNAALNISNPKLKSTKEEP

SEQ ID NO: 928 - protein, 726 aa, synthetic construct
SEVEFSHEYWMRHALSLAKRARDEREVPVGAVLVLNNRIIGVGWNRAIGLHDPTAHAEIMALRQGGLVMQNYRLTDATLYVTFEPCVMCAGAMVHSRIGRVVFGVRNSKRGAAGSLMNVLNYPGVNHCVEITEGILVDECAALLCDFYRMPRQVLNAQRKAQSSISSGGSSGGCSGSEMPGASESVTPKSSGGSSAGSTKNTITKTLKLRIVRPYNSAEVEKIVADEKNSREKIALERNKDKVKEACSEHLKVAAYCTTQVERNACLFCKARKLDDRFYQKLRGQFPDAVFWQETGEIFRQLQRQAAEIYNQSLIELYYEIFIKGKGFANASSVEHYLSDVCYTRAAELFKNAAIASGLRGKVKSNFRLKELKNMKSGLPTTKSDNFPIPLVKQKGGQYTGFEISSHNDDFIIKIPFGRWQVKKEIDKYRPWEKFDFEQVRKSPKPISLLLSTQRRKRNRGWSKDEGTEAEIRKVMNGDYQTSYIEVKRGSKIGEKSAWMLSLSIDVPKIDKGVDPSIIGGIDVGVKSPLVCAINNAFCRYSISDNDLFHFNKKMFARRRILLKKSRHKRAGHGAKNKLKPISILTEKSKRFRKKLIERWACEIADFFIKNKVGTVQMENLESMKRKEDSYFNIRLRGFWPYAEMQNKIEFKLKQYGIEIRKVAPNNTSKTCSKCGHLNNYFNFEYRRTNKFPHFKCEKCNFKEDADYNAALNISNPKLKSTKGEP

SEQ ID NO: 929 - protein, 726 aa, synthetic construct
SEVEFSHEYWMRHALTLAKRARDEREVPVGAVLVLNNRVIGEGWNRAIGLNDPTAHAEIMALRQGGLVMQNYRLIDATLYVTFEPCVMCAGAMIHSRIGRVVFGVRNNKHGAAGSLMNVLNYPGMNHRVEITEGILADECAALLCDFYRMPRQVFNARKKAQSSINPGGSSGGSGGSETPGTSESATPENSGGSSGSSAKNTITKTLKLRIVRPYNSAEVEKIVADEKNNRERIALEKNKDKVKEACSKHLKVAAYCTTQVERNACQFCKARKLDDKFYQKLRGQFPDAVFWQEIGEIFRQLQRQAAEIYNQSLIELYYEIFIKGRGFANASSVEHYLSDVCYTRAAELFKNAAIASGLRGKVKSNFRLKELKNMKSGLPTTKSDNFPIPLVKQKGGQYTGFEISSHNDDFIIKIPFGRWQVKKEIDKYRPWEKFDFGQVRKSPKPISLLLSTQRRKRNKGWNKDEGTEAEIRKVMNGDYQTSYIEVKRGSRIGEKSAWMLNLSIDVPKIDKGVDPSIIGGIDVGVKSPLVCAINNAFSRYSISDNDLFHFNKKMFARRRILLKKNRHKRAGHGAKNKLKPISILTEKSKRFRKKLIERWACEIADFFIKNKVGTVQMENLESMKRKEDSYFNIRLRGFWPYAEMQNKIEFKLKQYGIEIRKVAPNNTSKTCSKCGHLNNYFNFEYRKKNKFPHFKCEKCNFKENADYNAALNISNPKLKNTKEEP

SEQ ID NO: 930 - protein, 726 aa, synthetic construct
SEVEFSHEYWMRHALTLAKRARDEREVPVGAILVLNNRVIGEGWNRAIGLHDPTAHAEIMALRQGGLVMQNYRLTDATLYVTFEPCVMCAGAMIHSRIGRVVFGVRNSKRGAAGSLMNVLNYPGMNHRVEVTEGILADECAALLCDFYRMPRQVFNAQKKARSNINSGGSSGGSSGSEMPGTSESATPESSGGSSGGSARNTITKTLKLRIVRPYNSAEVEKIVADEKNNREKIALEKNKDKVKEACSEHLKVAAYCTTQVERNACLFCKARKLDDKFYQKLRGQFPDAVFWQEVGGIFRQLQKQAAEIYNQSLIELYYEIFIKGKGFANASSVEHYLSDVCYTRAAELFKNAAIASGLRGKVKSNFRLKELRSMRSGLPTTKSDNFPIPLVRQKGGQYTGFEISNHDGDFIIKIPFGRWQVKKEINKHRPWEKFDFEQVRKSPRPISLLLSTQRRKRNKGWSKDEGTEAEIRKVMNGDYQTSYIEVKRGSKIGEKSAWMLNLSIDVPKIDKGVDPRIIGGIDVGVKSPLVCAINNVLSRYSISDNDLFHFNKKMFARRRILLKKNGHKRAGHGAKNKLKPITIMTEKSKRFRKKLIERWACEIADFFIKNKVGTVQMENLESMKRKEDSYFNIRLRGFWPYAEMQSRIEFKLKQYGIEIRKVAPNNTSKTCSKCGHLNNYFSFEYRKKNKFPHFKCEKCNFKEDADYNAALNISNPKLKSTKEEP

SEQ ID NO: 931 - protein, 726 aa, synthetic construct
SEVEFSHEYWMRHALTLAKRARDEREVPVGAVLVLNNRVIGEGWNRAIGLHDPTAHAEVMALRQGGLVMQNYRLTDATLYVTFEPCVMCAGAMIHSRIGRVVFGVRNSKRGAAGSLVNVLNHPGMNHCVEITEGILVDECAALLCDFYRMPRQVLNAQKKAQSSISPGDSSGGSSGSEAPGASGSVTPKGSGGSSAGSTKDTITKTLKLRIVRPYNSAEVEKIVADEKNSREKIALEKNKDKVKEACSEHLKVAAYCTTQVERNACLFCKARKLDDRFYQKLRGQFPDAVFWQELGEIFRQLQKQAAEIYNQSLIELYYEIFIKGKGFANASSVEHYLSDVCYTRAAELFKNAAIASGLRGKVKSNFRLKELKNMKSGLPTTKSDNFPIPLVKQKGGQYTGFEISSHNDDFIIKIPFGRWQVKKEINKYRPWEKFDFEQVRKSPKPISLLLSTQRRKRNKGWSKDEGTEAEIRKVMNGDYQTSYIEVKRGSKIGEKSAWMLNLSIDVPKIDKGVDPSIIGGIDVGVKSPLVCAINNAFCRYSISDNDLFHFNKKMFARRRILLKKSRHKRAGHGAKNKLKPISILTEKSKRFRKKLIERWACEIADFFIKNKVGTVQMENLESMKRKEDSYFNIRLRGFWPYAEMQNKIEFKLKQYGIEIRKVAPNNTSKTCSKCGHLNNYFNFEYRKMNKFPHFKCEKCNFKENADYNAALNICNPKLKGTKEEP

SEQ ID NO: 932 - protein, 726 aa, synthetic construct
SEVEFSHEYWMRHALTLAKRARGEREVPVGAILVLNNRVIGEGWNRAIGLHDPTAHAEIMALRQGGLVMQNYRLIDATLYVTFEPCVMCAGAMIHSRIGRVVFGVRNSKHGAAGSLVNVLNYPGMNHRVEITEGILADECAALLCDFYRMPRQVFNARKKAQSSISPGGSSGGSSGSETPDASESVTPKSSGGSSGGSAKNTITKTLKLRIVRPYNSAEVEKIVADEKNNREKIALEKNKGKVKEACSKHLEVAAYCTTQVERNACLFCKARKLDDKFYQKLRDQFPDAVFWQEIGEIFRQLQKQAAEIYNQSLIELYYEIFIKGKGFANASSVEHYLSDVCYTRAAELFKNAAIASGLRGKVKSNFRLKELKNMKSGLPTTKSDNFPIPLVKQKGGQYTGFEISGHNDDFIIKIPFGRWRVKKEIDKYRPWEKFDFEQVRKSPKPISLLLSTQRRKRNKGWSKDEGTEAEIRKVMNGDYQTSYIEVKRGSKIGEKSAWMLNLSIDVPKIDKGVDPSIIGGIDVGVKSPLVCAINNAFSRYSISDNDLFHFNKKVFARRRILLKKNRHKRAGHGTKNKLKPITILTEKSGRFRKKLIERWACEIANFFIKNKVGTVQMENLESMKRKEDSYFNIRLRGFWPYAEMQNKIEFKLKQYGIKIRKVAPNNTSKTCSKCGHLNNYFSFEYRKKNKFPHFKCEKCNFKEDADYNAALNISNPKLKSTKEEP

SEQ ID NO: 933 - protein, 726 aa, synthetic construct
SEVEFSHEYWMRHALTLAKRARDGREVPVGAVLVLNNRVIGEGWNRAIGLHDPTAHAEIMALRQGGLVMQNYRLIDATLYVTFEPCVMCAGAMIHSRIGRVVFGVRNSKHGAAGSLVNVLNYPGMNHRVEITEGILVDECAALLCDFYRMPRQVFGARRKAQSSINPGGSSGGSSSSETPGTSESPTPESPGGSSGGSAKNTITKTLKLRIVRPYNSAEVEKIVADEKNNREKIALEKNKDKVKEACSKHLKVAAYCTTQVERNACLFCKARKLDDKFYQKLRGQFPDAVFWQEIGEIFRQLQKQAAEIYNQSLIELYYEIFIKGRGFANASSVEHYLSGVCYTRAAELFKNAAIASGLRGKVKSNFRLKELKNMKSGLPTTKSDNFPIPLVKQKGGQYTGFEISSHNDDFIIKIPFGRWQVKKEIDKYRPWEKFDFEQVRKSPKPISLLLSTQRRKRNKGWSKDEGTEAEIRKVMNGDYQTSYIEVKRGRKTGEKSAWMLNLSIDVPKIDRGVDPSIIGGIDVGVKSPLVCAINNAFSRYSISDNDLFRYNKKMFARRRILLKKNRHKRAGHGAKNKLKPISILTEKSKRFRKKLIERWACEIADFFIKNKVGTVQMENLESMKRKEDSYFNIRLRGFWPYAEMQNKIEFKLKQYGIEIRKVAPNNTSRTCSKCGHLNNYFNFEYRKKNKFPHFKCEKCNFKEDADYNAALNISNPKLKSTKEEH

SEQ ID NO: 934 - protein, 726 aa, synthetic construct
SEVEFSHEYWMRHALTLAKRARDEREVPVGAILVLNNRVIGEGWNRAIGLHDPTAHAEIMALRQGGLVMQNYRLIDATLYVTFEPCVMCAGAMIHSRIGRVVFGVRNSKRGAAGSLMNVLSYPGMNHCVEITEGILVDECAALLCDFYRMPRQVLNAQKKAQSSISSGGSSGGINGSETPGASESATPKSSGGSSAGSAKNTITKTLKLRIVRPYNSAEVEKIVADEKNSREKAALEKNKDKVKEACSKHLKVAAYCTTQVERSACLFCRARKLDDKFYQKLRGQFPEAVFWQEIGEIFRQLQKQAAEIYNQSLIELYYEIFIKGKGFANASSVEHYLSDVCYTRAAELFKNAAIASGLRGKVKSNFRLKELKNMKSGLPTTKSDNFPIPLVKQKGGQYTGFEISSHNDDFIIKIPFGRWQVKKEIDKYRPWEKFDFEQVRKSPKPISLLLSTQRRKKNKGWSKDESTEAEIRRVMNGDYQTSYIEVKRGSKIGEKSAWMLNLSIDVPKIDKGVDPSIIGGIDVGVKSPLVCAINNAFSRYSISDNDLFRFNKKMFARRRILLKKNRHKRAGHGAKNKLKPITILTEKSGRFRKKLIERWACEIADFFVKNKVGTVQMENLESMKRKEDSYFNIRLRGFWPYAEMQNKIEFKLKQYGIEIRKVAPNNTSKTCSKCGHLNNYFNFEYRKKNKFPHFKCEKCNFKENADYNAALNISNPKLKSTKEEP

SEQ ID NO: 935 - protein, 726 aa, synthetic construct
SEVEFSHEYWMRRALTLAKRARDEREVPVGAVLVLNNRVIGEGWNRAIGLHDPTAHAEIMALRQGGLVMQNYRLTDATLYVTFEPCVMCAGAMIHSRIGRVVFGVRNNKHGAAGSLVNVLNYPGMNHRVEITEGILADECAALLCDFYRMPRQVFNAQKKARPNINSGGSSGGRSGSETPGTSESATPESSGGSSGGSARNTITKTLKLRIVRPYNSAEVEKIVADEKNNREKVALEKNKDKVREACSKHLKVAAYCTTQVERSACLFCKARRLDDKFYQKLRGQFPDAVFWQEIGEIFRQLQKQAAEIYNQSLVELYYEIFIKGKGIANASSVEHYLSDVCYTRAAELFKNAAIASGLRGKVKSNFRLKELKNMKSGLPTTKSDNFPIPLVKQKGGQYTGFEISSHNDDFIIKIPFGRWQVKKEIDKYRPWEKFDFEQVRKSPKPISLLLSTQRRKKNKGWSKDEGTEAEIRRVMNGDYQTSYIEVKRGSKIGEKSAWMLNLSIDVPKIDKGVDPSIIGGIDVGVKSPLVCAINNALSRYSISDNDLFHFNKKMFARRRILLRKNRHKRAGHGAKNKLKPITMMTEKSKRFRKKLIERWACEIADFFIKNKVGTVQMENLESMKRKEDSYFNIRLRGFWPYAEMQNKIEFKLKQYGIVVRKVAPNNTSKTCSKCGHLNNYFNFEYRKKNKFPHFKCEKCNFKEDADYNAALNISNPKLKSTKGEP

SEQ ID NO: 936 - protein, 726 aa, synthetic construct
SEVEFSHEYWMRHALTLAKRARDEREVPVGAILVLNNRVIGVGWNRAIGLHDPTAHAEIMALRQGGLVTQNYRLIDATLYVTFEPCVMCAGAMIHSRIGRVVFGVRNSKRGAAGSLMNVLNYPGMNHCVEITEGILVDECAALLCDFYHMPRQVLNAQKKAQSSISSGGSSGGSSGSETPGASESVTPKSSGGSSAGSTKNTITKTLKLRIVRPYNSAEVEKIVADEKNNREKIALEKNKDKVKEACSKHLKVASYCTTQVERNACPFCKARKLDDKFYQKLRGQFPDAVFWQELGEILRQLQKQAAEIYNQSLIELYYEIFIKGRGFANTSSVEHYLSDVCYTRAAELFKNAAIASGLRGKVKSNFRLKELKNMKSGLPTTKSDNFPIPLVKQKGGQYTGFEISSHNDDFIIKIPFGRWQVKKEIDKYRPWEKFDFEQVRKSPKPISLLLSTQRRKRNKGWSKDEGTEAEIRKVMNGGYQTSYIEVKRGSKIGEKSAWMLNLSIDVPKIDKGVDPSIIGGIDVGVKSPLVCAINNSFSRYSICDNDLFRFNKKMFARRRILLKKNRHKRAGHGAKNKLKPITILTKKSERFRKKLIERWACEIANFFIKNKVGTVQMEDLESMKRKEDSYFNIRLRGFWPYAEMQNKIEFKLKQYGIEIRKVAPNNTSRTCSKCGHLNDYFNFEYRKKNKFPHFKCEKCNFKEDADYNAALNISNPKLKSTKEEP

SEQ ID NO: 937 - protein, 726 aa, synthetic construct
SEVEFSHEYWMRHALTLAKRARDEREVPVGAVLVLNNRVIGEGWNRAIGLYDPTAHAEIMALRQGGLVMQNYRLTDATLYVTFEPCVMCAGAMIHSRIGRVVFGVRNSKRGAAGSLMNVLNYPGMNHCVEITEGILMDECAALLCDFYRMPRQVLNAQKKAQSSISSGGPSGGSSCSETPGASESVTPKSSGGSSTGSTKNTITKTLKLRIVRPYNSAEVEKIVADEKNSREKIALEKNKDKVKEACREHLKVAAYCTTQVERSACLFCKARKLDDRFYQKLRGQSPDAVFWQELGEIFRQLQKQAAEIYNQSLIELYYEIFIKGKGFANASSVEHYLSDVCYTRAAELFKNAAIASGLRNKIKSNFRLKELRNMKSGLPTTKSDNFPIPLVRQKGGRYTGFEISNHNGDFIIKIPFGRWQVKKEINKHRPWEKFDFEQVRKSPKPISLLLSTQRRKRNKGWSKDEGTEAEIRKVMNGDYRTSYIEVKRGNKIGEKSAWMLNLSIDVPKIDKGVDPSIIGGIDVGVKSPLVCAINNAPSRYSISDNDLFHFNKKVFARRRILLKKNRHKRAGHGARNKLKPITVLTEKSERFRKKLIERWACEIAYFFIKNKVGTVQMEDLESMKRKEDSYFNIRLRGFWPYAEMQNKIEFKLKQYGIEVRKVAPNNTSKTCSKCGHLNSYFNFEYRKKNKFPHFKCEKCNFKEDADYNAALNISNPKLKSTKEEP

SEQ ID NO: 938 - protein, 726 aa, synthetic construct
SEVEFSHEYWMRHALTLAKRARDEREVPVGAVLVLNNRVIGEGWNRAIGLHDPTAHAEIMALRQGGLVMQNYRLSDATLYVTFEPCVMCAGAMVHSRIGRVVFGVRNSKRGAAGSLMNVLNYPGMNHRVEITEGILADECAALLCDFYRMPRQVFNAQKKAQSCINSGGSSGGSSGSDTPGTSESATPESSGGGSSGSAKNTITKTLQLRIVRPYNSAEVEKIVADEKNNREKIALEKNKDKVREACSKHLKVASYCTTQVERNACPFCKARKLDDKFYQKLRGQFPDAVFWQELGEILRQLQKQAAEIYNQSLIELYYEIFIKGKGFANASSVEHYLSDVCYTRAAELFKNAAIASGLRGKVKSNFRLRELKNMKSGLPTTKSDNFPIPLVKQKGGQYTGFEISNHNSDFIIKIPFGRWQVKKEVNKYRPWEKFDFEQVRKSPKPISLLLSTQRRKRNKGWNKDEGTEAEIRKVMNGDYQTSYVEVKRGSRIGEKSAWMLSLSIDVPKIDRGVDPSIIGGIDVGVKSPLVCAINNALSRYSISDNDLFHFNKKMFARRRILLKKNGHKRAGHGAKNKLKPITIMTEKSKRFRKKLIERWACEIADFFIKNKVGTVQMENLESMKRKEDSYFNIRLRGFWPYAEMQNKIEFKLKQYGIVIRKVAPNNTSKTCSKCGHLNNYFNFEYRKKNKFPHFKCEKCNFKENADYNAALNISNPKLKSTKEGP

SEQ ID NO: 939 - protein, 726 aa, synthetic construct
SEVEFSHEYWMRHALTLAKRARDEREVPVGAVLVLNNRVIGEGWNRTTGLHDPTAHAEIMALRQGGLAMQNYRLVDATLYVTFEPCVLCAGAMVHSRIGRVVFGVRNSKRGAAGSLMNVLNYPGMNHRVEITEGILADECAALLCDFYRMPRQVFNARKKARSNINSGGSSGGSSGSETLGTREGATPESSGGGSSGSAKNTITKTLQLRIVRPYNSAEVEKIVADEKNNREKIALEKNKDKVKEACSKHLKVASYCTTQVERSACPFCKARKLDDKFYQKLGGQFPDAVFWQELGEILRQLQKQAAEIYNQSLIELYYEIFIKGRGFANASSVEHYLSDVCYTRAAELFKNAAIASGLRGKVKSNFRLKELKNMKSGLPTTKSDNFPIPLVKQKGGQYTGFEISSHNDDFIIKIPFGRWQVKKEINKYRPWEKFDFEQVRKSPKPISLLLSTQRRKRNKGWGKDEGTEAEIRRVMNGNYQTSYIEVKRGSKIGEKSAWMLNLSIDVPKIDKGVDPSIIGGIDVGVKSPLVCAINNAFSRYSISDNDLFHFNKKMFARRRILLKKNRHKRAGHGAKNKLKRITILTEKSKRFRKKLIERWACEIADFFIKNKVGIVQMENLESMKRKEDSYFNIRLRGFWPYAEMQNRIEFKLKQYGIVVRKVAPNNTSKTCSKCGHLNNYFNFEYRKKNKFPHFKCEKCNFKEDADYNAALNISNPKLKSTKGEP

SEQ ID NO: 940 - protein, 726 aa, synthetic construct
SEVEFSHEYWMRRALTLAKRARDEREVPVGAVLVLNNRVIGVGWNRAIGLHDPTAHAEIMALRQGGLVTQNYRLIDATLYVTFEPCIMCAGAMIHSRIGRVVFGVRNSKRGAAGSLMNVLDYPGMNHRVEITEGILVDECAALLCDFYRMPRQVLNAQKKAQSSISPGGSSGGSSGSETPGASESVTPKSSGGSSGGSAKNTITKTLRLRIVRPYNSAEVEKIVADEKNNREKIALEMNKGKVKEACSEHLKVAAYCTTQVERNACLFCRARKLDDKFYQKLRGQFPDAVFWQEIGEIFRQLQKQAAEIYNQSLIELYYEIFIKGKGFANASSVEHYLSDVCYTRAAELFKNAAIASGLRGKVKSNLRLKELKNMKSGLPTTKSDNFPIPLVKQKGGQYTGFEISSHNDDFIIKIPFGRWQVKKEIDKYRPWEKFDFEQVRKSPKPISLLLSTQRRKRNKGWGKDEGTEAEIRKVMNGDYQTSYIEVKRGSKIGEKSAWMLSLSIDVPKIDKGVDPRIIGGIDVGVKSPLVCAINNALSRYSISDNDLFRFNKKMFARRRILLKKNRHKRAGHGAKNKLKPISILTEKSKRFRKKLIERWACEIADFFIKNKVGTVQMENLESMKRKEDSYFNIRLRGFWPYAEMQNKIEFKLKQYGIEIRKVAPNNTSKTCSKCGHLNNYFNFEYRKKNKFPHFKCEKCNFKENADYNAALNISNPKLKSTKEEP

SEQ ID NO: 941 - protein, 726 aa, synthetic construct
SEVEFSHEYWMRHALTLAKRARDEREVPVGAILVLNNRVIGEGWNRAVGLHDPTAHAEIMALRQGGLVMQNYRLIDATLYVTFEPCVMCAGAMIHSRIGRVVFGVRNSKHGAAGSLMNVLNYPGMNHRVEITGGILADECAALLCDFYRMPHQVFNARKKAQSSINPGGPSGGSSGSETPGTSESATPESSGGSSGGSTRNTITKTLQLRIVRPYNSAEVEKIVTDEKNNREKIALEKNKDKVKEACSKHLKMASYCTTQVERNACLFCKARKLDDKFYQKLRGQFPDAVFWQELGGILRQLQKQAAEIYNQSLIELYYEVFIKGRGFANASSVEHYLSDVCYTRAAELFKNAAIASGLRGKVKSNFRLKELKNMRSGLPTTKSDNFPIPLVKQKGGQYTGFEISSHNDDFIIKIPFGRWQVKKEIDKYRPWEKFDFEQVRKSPKPISLLLSTQRRKRSKGWSKDEGTEAEIRKVMNGDYQTSYIEVKRGSKTGEKSTWMLNLSIDVPKIDKGVDPSIIGGIDVGVKSPLVCAINNAFSRYSISDNDLFRFNKKMFARRRILLKKNRHKRAGHGAKNKLKPISILTGKSERFRKKLIERWACEIADFFIKNKVGTVQMENLESMKRKEDSYFNIRLRGFWPYAEMQNKIEFKLKQYGIEIRKVAPNNTSKTCSKCGHLNNYFNFEYRKKNKFPHFKCEKCNFKENADYNAALNISNPKLKSTKEEP

SEQ ID NO: 942 - protein, 726 aa, synthetic construct
SEVEFSHEYWMRHALTLAKRARDEREVPVGAVLVLNNRVIGEGWNRAIGLHDPTAHAEIMALRQGGLVMQNYRLIDATLYVTFEPCVMCAGAMVHSRIGRVVFGVRNSKRGAAGSLMNVLDYPGMGHRVEITEGILADECAALLCDFYCMPRQVFNAQKRAQSSINSGGSSGGSSGSETPGTSESATPESSGGGSSGSAKNTITKTLQLRIVRPYNSAEVEKIVADEKNNREKIALEKNKDKVKEACSKHLKVAAYCTTQVERNACLFCKARRLDDKFYQKLRGQFPDAVFWQEIGEIFRQLQKQAAEIYNQSLVELYYEILIKGKGIANASSVEHYLSDVCYTRAAKLFKNAAIASGLRNKIKSNFRLKELRNMKSGLPTTKSDNFPIPLVRQKGGQYTGFEISNHDGDFIIKIPFGRWQVKKEINKHRPWEKFDFEQVRKSPKPISLLLSTQRRKRNKGWSKDEGTEAEIRKVMNGDYQISYIEVKRGSKIGEKSAWMLNLSVDVPKIDKGVDPSIVGGIDVGVKSPLVCAINNALSRYSISDNDLFHFNKKMFARRRILLRKNRYKRAGHGARNKLKPITALTEKSERFRKKLIERWACEIANFFIKNKVGTVQMENLESMKRKEDSYFNIRLRGFWPYAEMQNKIEFKLKQYGIEIRRVAPNNTSRTCSKCGHLNNYFSFEYRKKNKFPHFKCEKCDFKENADYNAALNISNPKLKSTKEEP

SEQ ID NO: 943 - protein, 726 aa, synthetic construct
SEVEFSHEYWMRHALTLAKRARDEREVPVGAILVLNNRVIGEGWNRAIGLHDPTAHAEIMALRQGGLVMQNYRLIDATLYVTFEPCVMCAGAMIHSRIGRVVFGVRNNKHGAAGSLVNVLNYPGMNHRVGITEGILADECAALLCDFYRMPRQVFNARKKAQSSINPGGSSGGSSGSETPGTSESATPESSGGSSGGSAKNTITKTLKLRIVRPYNSAEVEKIVADEKNNREKIALEKNKDKVKEACSKHLKVAAYCTTQVERNACLFCKARRLDDKFYQKLRGQFPDAVFWQEIGEIFRQLQKQAAEIYNQSLIELYYEIFIKGKGFANASSVEHYLSDVCYTRAAELFKNAAIASGLRGKVKSNFRLKELKNMKSGLPTTKSDNFPIPLVKQKGGQYTGFEISNHNDDLIIKIPFGRWQVKKEIDKYRPWEKFNFEQVRKSPKPISLLLSTQRRKRNKGWSKDEGTEAEIRKVMNGDYQTSYIEVKRGSKIGEKSAWMLSLSIDVPKIDKGVDPSIIGGIDVGVKSPLVCAINNAFNRYSISDNNLFHFNKKMFARRRILLKKNRHKRAGHGAKNKLKPISILTEKSERFRKKLIERWACEIADFFIRNKVGTVQMENLEGMKRKEDSYFNIRLRGFWPYAEMQNKIEFKLKQYGIKIRKVAPNNTSKTCSKCGHLNNYFSFEYRKKNKFPHFKCEKCNFKENADYNAALNISNPKLKSTKEEP

SEQ ID NO: 944 - protein, 726 aa, synthetic construct
SEVEFSHEYWMRHALTLAKRARDEREVPVGAILVLNNRVIGEGWNRAIGLHDPTAHAEIMALRQGGLVMQNYRLIDATLYVTFEPCIMCAGAMIHSRIGRVVFGVRNSKRGAAGSLMNVLDYPGMGHRVEITEGILADECAALLCDFYCMPRQVFNAQKRAQSSINSGGSSGGSSGSETPGTSESATPESSGCGSSGSAKNTITKTLQLRIVRPYNSAEVEKIVADEKNNREKIALEKNKDKVKEACSKHLKVAAYCTTQVERNVCLFCKARKLDDKFYQKLRGQFPDAVFWQEIGEIFRQLQKQAAEIYNQSLIELYYEIFIKGRGFANASSVEHYLSDVCYTRAAELFKNAAIASGLRGKVKSNFRLKELKNMKSGLPTTKSDNFPIPLVKQKGGQYTGFEISSHNDDFIIKIPFGRWQVKKEINKFRPWEKFDLEQVRKSPKPISLLLSTQRRKRNKGWSRDEGTEAEIRKVMNGDYQTSYIEVKRGSKTGEKSAWMLSLSIDVPKIDKGVDPSIIGGIDVGVKSPLVCAINNAFSRYSISDNDLFHFNKKMFARRRILLKRNRHKRAGHGAKNKLKPITILTEKSKRFRRKLIERWACEIANFFIKNKVGTVQMENLEGMKRKEDSYFNIRLRGFWPYAEMQKKIEFKLKQYGIEIRKVAPNNTSKTCSKCGHLNNYFNFEYRKKNKFPHFKCEKCNFKENADYNAALNISNPKLKSTKEEP

SEQ ID NO: 945 - protein, 726 aa, synthetic construct
SEVEFSHEYWMRHALTLAKRARDEREVPVGAVLVLNNRVIGEGWNRAIGLHDPTAHAEIMALHQGGLVMQNYRLIDATLYVTFEPCVMCAGAMIHSRIGRVVFGARNSKRGAAGSLMNVLSYPGMNHRVEITEGILADECAALLCDFYRMPRRVFNAQKKAQSSINSVGSSGGGSGSETPSTSESATPESSGGSSGGPVKNTITKTLKLRIVRPYNSAEVEKIVADEKNNREKIALEKNKDKVKEACSKHLKVAAYCTTQVERNACLFCKARKLDDKFYQKLRGQFPDAVFWQEVGEIFRQLQKQAAEIYNQSLIELYYEIFIKGKGFANASSVEHYLSDVCYTRAAELFKNAAIASGLRGKVKSNFRLKELKNMKSGLPTTKSDNFPIPLVKQKGGQYTGFEISNHNSDFIIKIPFGRWQVKKEIDKYRPWEKFDFEQVRKSPKPISLLLSTQRRKRNKGWSKDEGTEAEIRKVLNGDYQTSYIEVKRGSKTGEKSAWMLNLSINVPKIDKGVDPSIIGGIDVGVKSPLVCAINNAFSRYSISDNDLFRFNKKMFARRRILLKKNRHKRAGHGAKNKLKPISILTGKSERFRKKLIERWACEIADFFIKNKVGTVQMENLESMKRKEDSYFNIRLRGFWPYAEMQNKIEFKLKQYGIEIRKVAPNNTSKTCSKCGHLNNYFNFEYRKKNKFPHFKCEKCNFKENADYNAALNISNPKLKSTKEKP

SEQ ID NO: 946 - protein, 726 aa, synthetic construct
SEVEFSHEYWMRHALTLAKRARDGREVPVGAVLVLNNRAIGEGWNRAIGLHDPTAHAEIMALRQGGLVMQNYRLIDATLYVTFEPCVMCAGAMVHSRIGRVVFGVRNSKRGAAGSLMNVLDYPGMDHRVEITEGILADECAALLCDFYRMPHQVFNAQKKAQSSINSGGSSGGSSGSETPGTSESATPESSGGSSGGSAKNTITKTLQLRIVRPYNSAEVEKIVTDEKNNREKIALEKNKGKVKEACSKHLKMASYCTTQVERNACLFCKARKLDDKFYQKLRGQFPDAVFWQELGGIFRQLQKQAAEIYNQSLIELYYEIFIKGKGITNASRVEHYLSDVCYTRAAELFKNAAIASGLRSKVRSNFRLKELKNMKSGLPTTKSDNFPIPLVKQKGGQYTGFEISSHNSDFIIKIPFGRWQVKEEIDKYRPWEKFDFEQVRKSPKPISLLLSTQRRKKNKGWSKDEGTEAEIRRVMNGDYQTSYIEVRRGSKIGEKSAWMLSLSIDVPKIDKGVDPSIIGGIDVGVKSPLVCAINNSFSRYSICDNDLFRFNKKMFARRRILLKRNRHKRAGHGAKNKLKPITILTKKSERFRKKLIERWVCEVADFFIKNKVGTVQMENLESMKRKEDSYFNIRLRGFWPYAEMQNKIEFKLKQYGIKIRKVAPNNTSKTCSKCGHLNNYFSFEYRKKNKFPHFKCERCNFKEDADYNAALNISNPKLKSTKEEP

SEQ ID NO: 947 - protein, 726 aa, synthetic construct
SEVEFSHEYWMRHALTLAKRARDEREVPVGAVLVLNNRVIGEGWNRAIGLHDPTAHAEIMALRQGGLVMQNYRLVEATLYVTFEPCIMCAGAMIHSRIGRVVFGVRNSKRGAAGSLMNVLNYPGMNHRVEITEGILADECAALLCDYYRMPRQVFNARKKALSSINSGGSSDGGSGSETPGTSESATPESSGGSSGGSAKNTITKTLKLRIVRPYNSAEVEKIVADEKNNREKIALEKNKDKVKEACSEHLKVAAYCTTQVERSACLFCKARKLDDKFYQKLRGQFPDAVFWQEIGEIFRQLQKQAAEIYNQSLIELYYEIFIKGKGFANASSVEHYLSDVCYTRAAELFKNAAIASGLRGKVKSNFRLKELKNMKSGLPTTKSDNFPIPLVKQKGGQYTGFEISSHNDDFIIKIPFGRWQVKKEIDKYRPWEKFDFEQVRKSPKPISLLLSTQRRKRNKGWSKDEGTEAEVRKVMNGDYRTSYIEVKRGSKIGEKSAWMLNLSIDVPKIDKGVDPSIIGGIDVGVKSPLVCAINNAFSRYSISDNDLFHFNKKMFARRRILLKKNGHKRAGHGAKNKLKPIAIMTEKSKRFRKKLIERWACEIADFFIKNKVGTVQMEDLESMKRKEDSYFNIRLRGFWPYAEMQNKIEFKLKQYGIVVRKVAPNNTSKTCSKCGHLNNYFNFEYRKKNKFPHFKCEKCNFKEDADYNAALNISNPKLKSTKGEP

SEQ ID NO: 948 - protein, 726 aa, synthetic construct
SEVEFSHEYWMRHALTLAKRARDEREVPVGAILVLNNRVIGEGWNCAIGLHDPTAHAEIMALRQGGLVMQNYRLIDATLYVTFEPCVMCAGAMIHSRIGRVVFGVRNSKRGAAGSLMNVLNYPGMNHRVEITEGILADECAALLCDFYRMPRRVLNARKKAQSNINSGGPSGGSSSSETPGTSESPTSEGSGGSSDGSAKNTITKTLKLRIVRPYNSAEVEKIVADEKNNREKIALEKNKDKVKEACSKHLKVAAYCTTQVERNACPFCKARKLDDKFYQKLRGQFPDAVFWQELGEILRQLQKQAAEIYNQSLIELYYEIFIKGRGFANASSVEHYLSDVCYTRAAELFKNAAIASGLRGKVKSNFRLKELKNMKSGLPTTKSDNFPIPLVKQKGGQYTGFEVSSHNDDFIIKIPFGRWQVKKEIDKYRPWEKFDFEQVRKSPKPISLLLSTQRRKRNKGWSKDEGTEAEIRKVMNGDYQTSYIEVKRGSKIGEKSAWMLNLSIDVPKIDKGVDPSVIGGIDVGVKSPLVCAINNAFSRCSISDNDLFHFNKKMFARRRILLKKNRHKRAGHGAKNKLKPITILTEKSKRFRKKLIERWACEIADFFIKNKVGTVQMENLESMKRREDSYFNIRLRGFWPYAEMQSKIEFKLKQYGIKIRKVAPNNTSKTCSKCGHLNNYFNFEYRKKNKFPHFKCEKCNFKENADYNAALNISNPKLKSTKEEP

SEQ ID NO: 949 - protein, 726 aa, synthetic construct
SEDEFSHEYWMRHALTLAKRARDGREVPVGAVLVLNNRVIGEGWNRAIGLHDPTAHAEIMALRQGGLVMQNYRLIDATLYVTFEPCVMCAGAMIHSRIGRVVFGVRNSKHGAAGSLVNVLNYPGMNHRVEITEGILAGECAALLCDFYRMPRQVFGARRKAQSSINPGGSSGGSSGSETPGTSESPTPESPGGGSSGSAKNTITKTLQLRIVRPYNSAEVEKIVADEKNNREKIALEKNKDKVKEACSKHLKVASYCTTQVERNACPFCKARKLDDKFYQKLRDQFPDAVFWQELGEILRQLQKQAAEIYNQSLIELYYEIFIKGRGFANASSVEHYLSDVCYTRAAELFKNAAIASGLRGKVKSNFRLKELKNMKSGLPTTKSDNFPIPLVKQKGGQYTGFEISSHNDDFIIKIPFGRWQVKKEIDKYRPWEKFDFEQVRKSPKPISLLLSTQRRKRNKGWSKDEGTEAEIRKVMNGDYQTSYIEVKRGSKIGEKSAWMLNLSIDVPKIDKGVDPSIVGGIDVGVKSPLVCAINNAFSRYSISDNDLFRFNKKMFARRRILLGKNRHKRAGHGVKNKLKPITILTEKSGRFRKKLIERWACEIADFFVKNKVGTVQMENLESMKRKEDSYFNIRLRGFWPYAEMQNKIEFKLKQYGIEIRKVAPNNTSKTCSKCGHLNNYFNFEYRKKNKFPHFKCEKCNFKENADYNAALNISNPKLKSTKEEP

SEQ ID NO: 950 - protein, 726 aa, synthetic construct
SEVEFSHEYWMRHALTLAKRARDEREVPVGAVLVLNNRVIGEGWNRAIGLHDPTAHAEIMALRQGGLVMQNYRLTDATLYVTFEPCVMCAGAMIHSRIGRVVFGVRNSKRGAAGSLMNVLNYPGMNHCVEITEGILVDECAALLCDFYRMPRQVFNARKKAQSSTNSGGSSDGGSGCETPGTSESATPESSGGSSGGSAKNTITKTLKLRIVRPYNSAEVEKIVADEKSNREKIALEKNKDKVKEACSKHLKVAAYCTTQVERNACLFCRARRLDDKFYQKLRGQFPDAVFWQEIGEIFRQLQKQAAEVYNQSLVELYYEILIKGKGIANASSVEHYLSNVCYTRAAELFKNAAIASGLRNKIKSNFRLKELRNMKSGLPTTKSDNFPIPLVRQKGGQYTGFEISSHNSDFIIKIPFGRWQVKEEIDKYRPWEKFDFEQVRKSPKPISLLLSTQRRKKNKGWSKDEGTEAEIRKVMNGDYQTSYIEVKRGSKIGEKSAWMLNLSIDVPKIDRGVDPSIIGGIDVGVRSPLVCAINNAFSRYSISDNDLFRFNKKMFARRRILLKKNRHKRAGHGAKNKLRPITILTEKSGRFRKKLIERWACEIANFFIKNKVGTVQMENLESMKRKEDSYFNIRLRGFWPYAEMQNKIEFKLKQYGIKIRKVAPNDTSKTCSKCGHLNNYFSFEYRRKNKFPHFKCEKCNFKEDADYNAALNISNPKLKSTKEEP

SEQ ID NO: 951 - protein, 726 aa, synthetic construct
SEVELSHEYWMRHALTLAKRARDEREVPVGAVLVLNNRVIGEGWNRAIGLHDPTAHAEIMALRQGGLVMQNHRLVNATLYVTFEPCVMCAGAMIHSRIGRVVFGVRNNKHGAAGSLVNVLDYPGMNHRVEITEGILADECAALLCDFYRMPRQVFNARKKAQSSISLGGSSGGSSGSETPGTSESATPESSGGSSGGSAKNTITKTLKLRIVRPYNSAEVEKIVADEKNSREKIALEKNKDKVKEACSEHLRVAAYCTTQVERDACLFCKARKLDDKFYQKLRGQFPDAVFWQETGEIFRQLQRQAAEIYNQSLIELYYEIFIKGKGFANASSVEHYLSDVCYTRAAELFKNAAIASGLRGKVKSNFRLKELKNMKSGLPTTKSDNFPIPLVKQKGGQYTGFEISSHNDDFIIKIPFGRWQVKKEIDKYRPWEKFDFEQVRKSPKPISLLLSTQRRKRNKGWSKDEGTEAEIRKVMNGDYQTSYIEVKRGSKIGEKSAWMLSLSIDVPKIDKGVDPSIIGGIDVGVKSPLVCAINNAFCRYSISDNDLFHFNKKMFARRRILLKKSRHKRAGHGAKNKLKPISILTEKSKRFRKKLIERWACEIADFFIKNKVGTVQMENLESMKRKEDSYFNIRLRGFWPYAEMQNKIEFKLKQYGIEIRKVAPNNTSKTCSKCGHLNNYFNFEYRKKNKFPHFKCEKCNFKENADYNAALNISNPKLKSTKEEP

SEQ ID NO: 952 - protein, 726 aa, synthetic construct
SEVEFSHEYWMRRALTLAKRARDEREVPVGAVLVLNNRVIGVGWNRAVGLHDPTAHAEIMALRQGGLVMQNYRLTDATLYVTFEPCVMCAGAMIHSRIGRVVFGVRNSKRGAAGSLMNVLNYPGMNHCVEITEGILVDECAALLCDFYRMPRQVLNAQKKAQPSISSGGSSGGSSGSETSGASESVTPKSSGGGSAGSTKNTITKTLKLRIVRPYNSAEVEKIVADEKNSREKIALEKNKDKVKEACSKHLKVAAYCTTQVERNACLFCKARKLDDKFYQKLRGQFPDAVFWQEIGEVFRQLQKQAAEIYNQSLIELYYEIFIKGRGFANASSVEHYLSDVCYTRAAELFKNAAIASGLRGKVKSNFRLKELKNMKSGLPTTKSDNFPIPLVKQKGGQYTGFEISSHNDDFIIKIPFGRWQVKKEIGKYRPWEKYDFEQVRKSPKPISLLLSTQRRKRNKGWSKDEGTEAEIRKVMNGDYQTSYIEVKRGSKTGEKSAWMLNLSIDVPKIDKGVDPSIIGGIDVGVKSPLVCAINNAFSRYSISDNDLFRFNKKMFARRRILLRKNRHKRAGHGAKNKLKPISILTGKSERFRKKLIERWACEIADFFIKNRVGTVQMENLESMKRKEDSYFNIKLRGFWPYAEMQNKIEFKLKQYGIEIRKVAPNNTSKTCSKCGHLNNYFNFEYRKKNKFPHFKCEKCNFKENADYNAALNISNPKLKSTKEEP

SEQ ID NO: 953 - protein, 726 aa, synthetic construct
SEVEFSHEYWMRHALTLAKRARDEREVPVGAVLVLNNRVIGEGWNRAIGLHDPTAHAEIMALRQGGLVMQNYRLIDATLYVTFEPCVMCAGAMIHSRIGRVVFGVRNSKHGAAGSLMNVLNYPGMNHRVEITGGILADECAALLCDFYRMPRQVFNAQKKARSNINSGGSSGGSSGSETLGTSESATPESSGGSSGGSAKNTITKTLKLRIVRPYNSAEVEKIVADEKNNREKIALEKNKDRVKEACSEHLKVAAYCTTQVERNACLFCKARKLDDKFYQKLRGRFPDAVFWQEISEIFRQLQKQAAEIYNQSLIELYYEIFIKGKGFANASSVEHYLSDVCYTRAAELFKNAAIASGLRGKVKSNFRLKELKNMKSGLPTTKSDNFPIPLVRQKGGQYTGFEISSHNDDFIIKIPFGRWQVKEEIDKYRPWEKFDFEQVRRNPKPISLLLSTQRRKRNKGWSKDEGTEAEIRKVMNGDYQTSYIEVKRGSKTGEKSAWMLNLSIDVPKIDKGVDPSIIGGIDVGVKSPLVCAINNAFSRYSISDNDLFRFNKKMFARRRILLKKNRHKRAGHGAKNKLKPISILTGKSERFRKKLIERWACEIADFFVKNKVGTVQMENLESMKGKEDSYFNIRLRGFWPYAEMQNKIEFKLKQYGIEIRKVAPNNTSKTCSKCGHLNNYFNFEYRKKNKFPHFKCEKCNFKENADYNAALNISNPKLKSTKEEP

SEQ ID NO: 954 - protein, 726 aa, synthetic construct
SEVEFSHEYWMRHALTLAKRARDEREVPVGAILVLNNRVIGEGWNRAIGLHDPTAHAEIMALRQGGLVMQNYRLIDATLYVTFEPCVMCAGAMIHSRIGRVVFGVRNNKHGAAGSLVNVLNYPGMNHRVEITEGILADECAALLCDFYRMPRQVFNARKKAQSSINPGGSSGGSSGSETPGTSESATPESSGGSSGGSAKNTITKTLQLRIVRPYNSAEVEKIVTDEKNNREKIALEKNKDKVKEACSKHLKMAPYCTTQVERNTCLFCKARKLDDKFYQKLRGQFPDAVFWQELGEIFRQLQKQAAEIYNQSLIELYYEIFIKGKGLANASSVEHYLSDVCYTRAAELFKNAAIASGLRGKVKSNFKLKELKSMKSGLPTTKSDNFPIPLVKQKGGQYTGFEISSHNDDFIIKIPFGRWQVKKEIDKYRPWEKFDFEQVRKSPKPISLLLSTQRRKRNKGWSKDEGTEAEIRKVMNGDYQTSYIEVKRGSKIGEKSAWMLSLSIDVPKIDKGVDPSIIGGIDVGVKSPLVCAINNAFGRYSISDNDLFRFNKKMFARRRILLKKNRHKRAGHGAKNKLKPITILTGKSERFRKKLIERWACEIADFFIKNKVGTVQMENLESMKRKEDSYFNIRLRGFWPYAEMQNKIEFKLKQYGIEIRKVAPNNTSKTCSKCGHLNNYFNFEYRKKNKFPHFECEKCNFKENADYNAALNISNPKLKSTKEEP

SEQ ID NO: 955 - protein, 726 aa, synthetic construct
SEVEFSHEYWMRHALTLAKRARDEREVPVGAILVLNNRVIGVGWNRAIGLHDPTAHAEIMALRQGGLVTQNYRLIDATLYVTFEPCVMCAGAMIHSRIGRVVFGVRNSKHGAAGSLVNVLNYPGMNHRVEITEGILADECAALLCDFYRMPRQVFNARKKAQSSTNPGGSSGGSSGSEAPGTSESATPESSGSSSGGSAKNTITKTLKLRIVRPYNSAEVEKIVADEKNNREKIALEKNKDKVKEACSKHLKVAAYCTTQVERNACPFCKARKLDDKFYQKLRGQFPDAVFWQEIGEIFRQLQKQAAEIYNQSLVELYYEIFIKGRGIANASSVEHYLSDVCYTRAAELFKNAAIASGLRNKIKSNFRLKELRNMKSGLPTTKSDNFPIPLVRQKGGQYTGFEISNHNSDFIIKIPFGRWQVKKEIDKYRPWEKFDFEQVRKSPKPISLLLSTQRRKRNKGWSKDVGTEAEIRKVMNGDYQTSYIEVKRGSKIGEKSAWMLNLSIDVPKIDKGVDPSIIGGIDVGVKSPLVCAINNAFSRYSISDNDLFHYNKKMFARRRILLKKNRHKRAGHGAKNKLKPISILTEKSKRFRKTLIERWACEIANFFIRNKVGTVQMENLEGMKRREDSYFNIRLRGFWPYAEMQNKIEFKLKQYGIEVRKVAPNNTSKTCSKCGHLNNYFNFEYRKKNKFPHFKCEECNFKENADYNAALNISNPKLKSTKEEP

SEQ ID NO: 956 - protein, 726 aa, synthetic construct
SEVEFSHEYWMRHALTLAKRARDEREVPVGAILVLNNRVIGEGWNRAIGLHDPTAHAEIMALRQGGLAMQNYRLTDATLYATFEPCVMCAGAMIHSRIGRVVFGVRNSKHGAAGSLMNVLNYPGMNHRVEITEGILADECAGLLCDFYRMPRQVFSARKKAQSSINPGGSSGGSSGGKAPGASGSVTPKSSGGSSAGSTKDTITKTLKLRIVRPYNSAEVEKIVADEKNNRERIALEKNKDKVKEACSKHLKVAAYCTTQVERNACLFCKARKLDDKFYQKLRGQYPDAVFWQELGEILRQLQKQAAEIYNRSLIELYYEIFIKGKGFANASSVEHYLSDVCYTRAAELFKNAAIASGLRSKVRSNFRLKELKNMKSGLPTTKSDNFPIPLVKQKGGQYTGFEISSHNDDFIIKIPFGRWQVKEEIDKYRPWEKFDFEQVRKNPKPISLLLSTQRRKRNKGWSKDEGTEAEIRKVMNGDYQTSYIEVKRGSKTGEKSAWMLNLSIDVPKIDKGVDPSIVGGIDVGVKSPLVCAINNALSRYSISDNDLFHFNKKMFARRRILLKKNRHRRAGHGAKNKLRPITILTEKSKRFRRKLIERWACEIADFFIKNKVGTVQMENLESMKRKEDSYFNIRLRGFWPYAEMQNKIEFKLKQYGIEIRKVAPNNTSKTCSKCGHLNNYFNFEYRKKNKFPHFKCEKCNFKESADYNAALNISNPKLKSTKGEP

SEQ ID NO: 957 - protein, 726 aa, synthetic construct
SEVEFSHEYWMRHALTLAKRARDEREVPVGAILVLNNRVIGEGWNRAIGLHDPTAHAEIMALRQGGLVMQNYRLIDATLYVTFEPCVMCAGAMIHSRIGRVVFGVRNSKHGAAGSLVNVLNYPGMNHRVEITEGILVDECAALLCDFYRMPRQVLNAQKKAQSSISSGGSSGGSSGSETPGTSESATPESSGGSSGGSAKNTITKTLKLRIVRPYNSAEVEKIVADEKSNREKIALEKNKDKVKEACSEHLKVAAYCTTQVERNACLFCKARKLDDKFYQRLRGQFPDAVFWQELGEIFRQLQKQAAEIYNQSLIELYYEIFIKGKGFANASSVEHYLSDVCYTRAAELFKNAAIASGLRGKVKSNFRLKELKNMKSGLPTTKSDNFPIPLVRQKGGQYTGFEISNHNGDFIIKIPFGRWQVKKEIDKYRPWEKFDFEQVRKSPKPISLLLSTQRRKRNKGWSKDEGTEAEIRKVMNGDYQTSYIEVKRGSKIGEKSAWMLNLSIDVPKIDKGVDPSIIGGIDVGVKSPLVCAINNAFSRYSISDNDLFHYNKKMFARRRILLKKNRHKRAGHGAKNKLKPISILTEKSKRFRKKLIERWACEIADFFIKNKVGTVQMENLESMKRKEDSYFNIRLRGFWPYAEMQNKIEFKLKQYGIEIRKVAPNNTSKTCSKCGHLNNYFNFEYRKMNKFPHFKCEKCNFKENADYNAALNISNPKLKSTKGEP

SEQ ID NO: 958 - protein, 726 aa, synthetic construct
SEVEFSHEYWMRHALTLAKRARDEREVPVGAVLVLNNRVIGEGWNRAIGLYDPTAHAEIMALRQGGLVMQNYRLIDATLYVTFEPCVMCAGAMVHSRIGRVVFGVRNSKRGAAGSLMNVLDYPGMGHRVEITEGILADECAALLCDFYCMPRQVFNAQKRAQSSINSGGSSGGSSGSETPGTSESATPESSGGSSGGSTKDTITKTLKLRIVRPYNSAEVEKIVADEKNSREKIALEKNKDKVKEACSEHLKVAAYCTTQVERNACLFCKARKLDDGFYQKLRGQFPDAVFWQEIGEIFRQLQKQAAEIYNRSLIELYYEIFIKGKGFANASSVEHYLSNVCYTRAAELFKNAAIASGLRGKVKSNFRLKELKNMKSGLPTTKSDNFPIPLVRQKGGQYTGFEISSHNDDFIIKIPFGRWQVKKEIDKYRPWEKFDFEQVRKSPKPISLLLSTRRRKKNKGWSKDEGTEAEIRKVMNGDYQTSYIEVKRGSKIGEKSAWMLNLSIDVPKIDKGVDPGIIGGIDVGVKSPLVCAINNASSRYSISDNDLFHFNKKMFARRRILLKKNRHKRAGHGAKNKLKPITIMTEKSKRFRKKLIERWACEIADFFIKNKVGTVQMENLESMKRKEDSYFNIRLRGFWPYAEMQNKIEFKLKQYGIEIRKVAPNNTSRTCSKCGHLNNYFNFEYRRKNKFPHFKCEKCNFKEDADYNAALNISNPKLKSTKEEP

SEQ ID NO: 959 - protein, 726 aa, synthetic construct
SEVEFSHEYWMRHALTLAKRARDEREVPVGAILVLNNRVIGEGWNRAIGLHDPTAHAEIMALRQGGLVMQNYRLIDATLYVTFEPCVMCAGAMIHSRIGRVVFGVRNSKRGAAGSLMNVLSYPGMNHCVEITEGILVDECAALLCDFYRMPRQVLNAQKKAQSSISSGGSSGGINGSETPGASESATPKSSGGSSAGSAKNTITKTLKLRIVRPYNSAEVEKIVADEKNSREKAALEKNKDKVKEACSKHLKVAAYCTTQVERSACLFCRARKLDDKFYQKLRGQFPEAVFWQEIGEIFRQLQKQAAEIYNQSLIELYYEIFIKGKGFANASSVEHYLSDVCYTRAAELFKNAAIASGLRGKVKSNFRLKELKNMKSGLPTTKSDNFPIPLVKQKGGQYTGFEISSHNDDFIIKIPFGRWQVKKEIDKYRPWEKFDFEQVRKSPKPISLLLSTQRRKKNKGWSKDESTEAEIRRVMNGDYQTSYIEVKRGSKIGEKSAWMLNLSIDVPKIDKGVDPSIIGGIDVGVKSPLVCAINNSSSRYSICDNDLFRFNKKMFARRRILLKKNRHKRAGHGAKNKLKPISILTEKSKRFRKKLIERWACEIADFFIKNKVGTVQMENLESMKRKEDSYFNIRLRGFWPYAEMQNKIEFKLKQYGIEIRKVAPNNTSKTCSKCGHLNNYFNFEYRKKNKFPHFKCEKCNFKEDADYNAALNISNPKLKSTKEEP

SEQ ID NO: 960 - protein, 726 aa, synthetic construct
SEAEFSHEYWMRHALTLAKRARDEREVPVGAILVLNNRVIGEGWNRAIGLHDPTAHAEIMALRQGGLVMQNYRLIDATLYVTFEPCVMCAGAMIHSRVGRVVFGVRNSKHGAAGSLMNVLNYPGMNHRVEITEGILADECAALLCDFYRMPRQVFNARKKAQSSINSGGSSGGSSGSETPGTSESATPKSSGGSSGGSAKNTITKALKLRIVRPYNSAEVEKIVADEKNNRERIALEKNKDKVKEACSKHLKVAAYCTTQVERNACLFCKARKLDDKFYQKLRGQFPDAVFWQEIGEIFRQLQKQAAEIYNQSLIELYYEILIKGKGFANASSVEHYLSDVCYARAAELFKNAAIASGLRGKVKSNFRLKELKNMRSGLPTTKSDNFPIPLVKQKGGQYTGFEISSHNDDFIIKIPFGRWQVKKEIDKYRPWEKFDFEQVRKSPKPISLLLSTQGRQKNKGWSKDEGTEAEIRRVMNGDYQTSYIEVKRGSKIGEKSTWMLNLSIDVPKIDKGVDPSIVGGIDVGVKSPLVCAINNSFSRYSICDNDLFRFNKKMFARRRILLKKNRHKRAGHGAKNKLKPISILTEKSKRFRKKLIERWACEIADFFIKNKVGTVQMENLESMKRKEDSYFNIRLRGFWPYAEMQNKIEFKLKQYGIEIRKVAPNNTSKTCSKCGHLNNYFNFEYRRKNKFPHFKCEKCNFKENADYNAALNISNPKLKSTKEEP

SEQ ID NO: 961 - protein, 726 aa, synthetic construct
SEVEFSHEYWMRHALTLAKRARDEREVPVGAILVLNNRVIGEGWNRAIGLHDPTAHAEIMALRQGGLVMQNYRLIDATLYVTFEPCVMCAGAMIHSRIGRVVFGVRNNKHGAAGSLVNVLNYPGMNHRVKITEGILADECAALLCDFYRMPHQVFNAQKKAQSSIDPGGPSGGSSGSETPGTSESATPESSGGSSGGSAKNTITKTLKLRIVRPYNSTEVEKIVADEKNNREKIALEKNKDKVKEACSKHLKVASYCTTQVERNACLFCKARKLDDKFYQKLGGQFPDAVFWQELGEIFRQLQKQAAEIYNQSLIELYYEIFIKGKGFANASSVEHYLSDVCYTRAAELFKNAAIASGLRGKVKSNFRLKELKNMKSGLPTTKSDNFPIPLVKQKGGQYTGFEISSHNGDFIIKIPFGRWQVKKEIDKYRPWEKFDFEQVRKSPKPISLLLSTQRRKRNKGWSKDEGTEAEIRKVMNGDYRTSYIEVKRGSKIGEKSAWMLNLSIDVPKIDKGVDPSIIGGIDVGVKSPLVCAINNSFSRYSISDNDLFHFNKKMFARRRILLKKNGHKRAGHGAKNKLKPIAIMTEKSKRFRKKLIERWACEIADFFIKNKVGTVQMENLESMKRKEDSYFNIRLRGFWPYAEMQNKIEFKLKQYGIEVRKVAPNNTSKTCSKCGHLNNYFNFEYRKKNKFPHFKCEKCNFKENADYNAALNISNPKLKSTKEEP

SEQ ID NO: 962 - protein, 726 aa, synthetic construct
SEVEFSHEYWMRHALTLAGRARDEREVPVGAVLVLNNRVIGEGWNRAIGLHDPTAHAEIMALRQGGLVMQNYRLIDATLYVTFEPCVMCAGAMIHSRIGRVVFGVRNSKHGAAGSLVNVLNYPGMNHRIEITEGILADECAALLCDFYRMPRQVFNARKKAQSSINSGGSSGGSSGSETPGTSESATPKNSGGSSGGSAKNTITKALKLKIVRPYNSAEVEKIVADEKNNRERIALEKNKDKVKEACCKHLKVAAYCTTQVERNACLFCKARKLDDKFYQKLRGQFPDAVFWQEIGEIFRQLQKQAAEIYNQSLIELYYEIFIKGKGFANASSVEHYLSDVCYTRAAELFKNAAIASGLRGKVKSNFRLKELKNMRSGLPTTKSDNFPIPLVKQKGGQYAGFEISSHNDDFIIKIPFGRWQVKKEIDKYRPWEKFDFEQVRKSPKPISLLLSTRRRKRNKGWSKDEGTEAEIRKVMNGDYQTSYIEVKRGSKIGEKSAWMLNLSIDVPKIDKGVDPSIIGGIDVGVKSPLVCAINNAFSRYSISDNDLFHFNKKMFARRRILLKKNRHKRAGHGAKNKLKPISTLTERSKRFRKKLIERWACEIADFFIKNKVGTVQMENLESMKRKEDSYFNIRLRGFWPYAEMQNKIEFKLKQYGIEIRKVAPNNTSKTCSKCGHLNNYFNFEYRKKNKFPHFKCEKCNFKENADYNAALNISNPKLKSTKKEP

SEQ ID NO: 963 - protein, 726 aa, synthetic construct
SEVEFSHEYWMRHALTLAKRARDEREVPVGAVLVLNNRVIGEGWNRAIGLHDPTAHAEIMALHQGGLVMQNYRLIDATLYVTFEPCVMCAGAMIHSRIGRVVFGARNSKRGAAGSLMNVLSYPGMNHRVEITEGILADECAALLCDFYRMPRRVFNAQKKAQSSINSGGSSGGGSGSETPSTSENTTPESSGGSSGGPAKNTITKTLKLRIVRPYNSAEVEKIVADEKNNREKTALERNKDKVKEACSKHLKVASYCTTQVERNACLFCKARKLDDKFYQKLRGQFPDAVFWQELGEIFRQLQKQAAEIYNQSLIELYYEIFIKGKGFANASSVEHYLSDVCYTRAAELFKNAAIASGLRGKVKSNFRLKELKNMKSGLPTTKSDNFPIPLVKQKGGQYTGFEISSHNDDFIIKIPFGRWQVKKEIDKYRPWEKFDFEQVRKSPKPISLLLSTQRRKRNKGWSKDEGTEAEIRKVMNGDYQTSYIEVKRGSKTGEKSAWMLNLSIDVPKIDKGVDPSIIGGIDVGVKFPLVCAINNAFSRYSISDNDLFRFNKKMFARRRILLKKNRHKRAGHGAKNKLKPISILTGKSERFRRKLIERWACEIADFFIKNKVGTVQMENLESMKRKEDSYFNIRLRGFWPYAEMQNKIEFKLKQYGIEIRKVAPDNTSRTCSKCGHLNNYFNFEYRKKNKFPHFKCEKCNFKENADYNAALNISNPKLKSTKEGP

SEQ ID NO: 964 - protein, 726 aa, synthetic construct
SEVEFSHEYWMRHALTLAKRARDEREVPVGAILVLNNRVIGEGWNRAIGLHDPTAHAEIMALRQGGLVMQNYRLTDATLYATFEPCVMCAGAMIHSRIGHVVFGVRNSKHGAAGSLMNVLNYPGMNHRVEITEGILADECAGLLCDFYRMPRQVFSARKKAQSNINSGGSSGGSSGSETPGTSESPTPESSGGSSGGSAKNTITKTLKLRIVRPYNSAEVEKIVADEKNNREKIALEKNKDKVKEACSKHLKVAAYCTTQVERNACLFCRARKLDDKFYQKLRGQFPDAVFWQEIGEIFRQLQKQAAEVYNQSLIELYYEIFIRGKGFANASSVEHYLSDVCYTRAAELFKNAAIASGLRGKVKSNFRLKELKNMKSGLPTTKSDNFPIPLVKQKGGQYTGFEISSHNDDFIIKIPFGRWQVKKEIDKYRPWEKFDFEQVRKSPKPISLLLSTRRRKRNKGWSKDEGTEAEIRKVMNGDYQTSYIEVKRGSKIGEKSAWMLSLSIDVPKIDKGVDPSIVGGIDVGVKSPLVCAIDNALSRYSISDNDLFHFNKKMFARRRILLKKNRHRRAGHGAKNKLKPISILTEKSKRFRKKLIERWASEIADFFIKNKVGTVQMENLESMKRKEDSYFNIRLRGFWPYAEMQNKIEFKLKQYGIEIRKVAPNNTSKTCSKCGHLNNYFNFEYRKKNKFPHFKCEKCYFKEDADYNAALNISNPKLKSTKEEP

SEQ ID NO: 965 - protein, 726 aa, synthetic construct
SEVEFSHEYWMRHALTLAKRARDEREVPVGAVLVLNNRVIGEGWNRAIGLHDPTAHAEIMALRQGGLVMQNYRLIDATLYVTFEPCVMCAGAMIHSRIGRVVFGVRNNKHGAAGSLVNVLNYPGMNHRVEITEGILADECAALLCDFYRMPRQVFIARKKAQSSINSGGSSGDSSGSETPGTSESATPKSSGGSSGGSAKNTITKALKLRIVRPYNSAEVEKIVADEKNNRERIALEKNKDKVKEACSKHLKVAAYCTTQVERNACLFCKARKLDDKFYQKLRGQFPDAVFWQEIGEIFRQLQKQAAEIYNQSLIELYYEIFIKGKGFANASSVEHYLSDVCYTRAAELFKNAAIASGLRGKVKSNFRLKELKNMRSGLPTTKSDNFPIPLVKQKGGQYAGFEICSHNDDFIIKIPFGRWQVKKEIDKYRPWEKFDFGQVRKSPKPISLLLSTRRRKRNKGWSKDEGTEAEIRKVMNGDYQTSYIEVKRGSKIGEKSAWMLSLSIDVPKIDKGVDPSIIGGIDVGVKSPLVCAINNAFGRYSISDNDLFHFNKKMFAMRRILLKKNRHKRAGHGAKNKLKPITILTEKSKRFRKKLIERWACEIADFFIKNKVGTVQMENLESMKRKEDSYFNIRLRGFWPYAEMQDKIEFKLKQYGIEIRKVAPNNTSKTCSRCGHLNNYFNFEYRRKNKFPHFKCEKCNFKENADYNAALNISNPKLKSTKEEP

SEQ ID NO: 966 - protein, 726 aa, synthetic construct
SEDEFSHEYWMRHALTLAKRARDGREVPVGAVLVLNNRVIGEGWNRAIGLHDPTAHAEIMALRQGGLVMQNYRLIDATLYVTFEPCVMCAGAMVHSRIGRVVFGVRNSKRGAAGSLMNVLNYPGMNHRVEITEGILVDECAALLCDFYRMPRQVFNAQKKAQSTINSGGSSGGSSGSETPGTSESPTPESSGGSPGGSAKNTITKTLQLRIVRPYNSAEVEKIVADEKNNREKIALEKNKDKVKEACSKHLMVASYCTTQVERNACPFCKARKLDDKFYQKLRGQFPDAVFWQELGEILRQLQKQAAEIYNQSLIELYYEIFIKGRGFANASSVEHYLSDVCYTRAAELFKNAAIASGLRGKVKSNFRLKELKNMKSGLPTTKSDNFPIPLVKQKGGQYTGFEISSHNDDFIIKIPFGRWQVKKEIDKYRPWEKFDFEQVRKCPKPISLLLSTQRRKRNKGWGKDEGTEAEIRKVMNGDYQTSYIEVKRGSKTGEKSAWMLNLSIDVPKIDKGVDPSIIGGIDVGVKSPLVCAINNAFSRYSISDNDLFRFNKKMFARRRILLKKNRHKRAGHGAKNKLKPISILTGKSERFRKKLIERWACEIADFFIKNKVGTVQMENLESMKRRGDSYFNIRLRGFWPYAEMQNKIEFKLKQYGIEIRKVAPNNTSKTCSKCGHLNNYFNFEYRKKNKFPHFKCEKCNFKENADYNAALNISNPKLKSTKEEP

SEQ ID NO: 967 - protein, 726 aa, synthetic construct
SEVEFSHEYWMRHALTLAKRARDEHEVPVGAVLVLNNRVIGEGWNRAIGLHDPTAHAEIMALRQGGLVMQNYRLIDATLYVTFEPCVMCAGAMIHSRIGRVVFGVRNSKHGAAGSLVNVLNYPGMNHRVEITEGILADECAALLCDFYRMPRQVFNARKKAQSSINPSGSSGGSSGSVTPGTSESATPESSGGGFGGSAKNTITKTLQLRIVRPYNSAEVEKIVADEKNNREKIALEKNKDKVKEACSKHLKVASYCTTQVERNACLFCKARKLDDKFYQKLRGQFPDAVFWQELGEIFRQLQKQAAEIYNQSLIELYYVIFIKGKGFANASSVEHYLSDVCYTRAAELFKNAAIASGLRGKVKSNFRLKELRNMKSGLPTTKSDNFPIPLVKQKGGQYTGFEISNHNSDFIIKIPFGRWQVKKEIDKYRPWEKFDFEQVRKSPKPISLLLSTQRRKRNKGWSKDEGTEAEIRKVMNGDYQTSYIEVKRGSKTGEKSAWMLNLSIDVPKIDKGVDPSIIGGIDVGVKSPLVCAINNAFSRYSISDNDLFRFNKKMFARRRILLRKNRHKRAGHGAKNKLKPISILTGKSERFRKKLIERWACEIADFFIKNKVGTVQMENLESMKRKEDSYFNIRLRGFWPYAEMQNKIEFKLKQYGIEIRKVAPNNTSKTCSKCGHLNNYFNFEYRKRNKFPHFKCEKCNYKEDADYNAALNISNPKLKSTKEGP

SEQ ID NO: 968 - protein, 726 aa, synthetic construct
SEVEFSHEYWMRHALTLAKRARDEREVPVGAVLVLNNRVIGEGWNRAIGLHDPTAHAEIMALRQGGLVMQNYRLIDATLYVTFEPCVMCAGAMIHSRIGRVVFGIRNNKHGAAGSLVNVLNYPGMNHCVEITEGILVDECAALLCDFYRMPRQVLNAQKKAQSSISPGGSSGGSSGSETPGASESVTPKSSGGSSGGSAKNTITKTLKLRIVRPYNSAEVEKIVADEKNNREKIALEKNKGKVKEACSKHLKVAAYCTTQVERNACLFCKARRLDDKFYQRLRGQFPDAVFWQEIGEIFRQLQKQAAETYNQSLVELYYEIFIKGKGIANASNVEHYLSDVCYTRAAELFKNAAIASGLRGKVKGNFRLKELKNMKSGLPTTKSDNFPIPLVKQKGGQYTGFEISSHNDDFIIKIPFGRWQVKKEIDKYRPWEKFDFEQVRKSPKPISLLLSTQRRRRNKGWGKDEGTEAEIRKVMNGDYQTSYIEVKRGSKTGEKSAWMLNLSIDVPKIDKGVDPSIIGGIDVGVKSPLVCAINNAFSRYSIGDNDLFRFNKKMFARRRILLKKNRHKRAGHGAKNKLKPITILTEKSRRFRKKLIERWACEIADFFIKNKVGTVQMESLESMKRKEDSYFNIRLRGFWPYAEMQNKIEFKLKQYGIKIRKVAPNNTSKTCSKCGHLNNYFSFEYRKKNKFPHFKCEKCNFKEDADYNAALNISNPKLKSTKEEP

SEQ ID NO: 969 - protein, 726 aa, synthetic construct
SEAEFSHEYWMRHALTLAKRARDEGEVPVGAILVLNNRVIGVGWNRAIGLHDPTAHAEIMALRQGGLVIQNYRLIDATLYVTFEPCVMCAGAMIHSRIGRVVFGVRNSKHGAAGSLVNVLNYPGMNHRVEITEGILADECAALLCDFYRMPRQVFNARKKAQSSINSGGSSGGSSGSETPGTSESATPKSSGGSSGGSAKNTITKALKLRIVRPYNSAEVEKIVADEKNNRERIALEKNKDKVKEACSKHLKVAAYCTTQVERNACLFCKARKLDDKFYQKLRGQFPDAVFWQEIGEIFRQLQKQAAEIYNQSLIELYYEILIKGKGFANASSVEHYLSDVCYTRAAELFKNAAIASGLRGKVKSNFRLKELKNMRSGLPTTKSDNFPIPLVKQKGGQYAGFEISSHNDDFIIKIPFGRWQVKKEIDKYRPWEKFDFEQVRKSPKPISLLLSTRRRKRNKGWSKDEGTEAEIRKVMNGDYQTSYIEVKRGSKIGEKSAWMLNLSIDVPRIDKGVDPSIIGGIDVGVKSPLVCAINNAFGRYSISDNDLFHFNKKMFARRRILLKKNRHKRAGHGAKNKLKPITILTEKSKRFRKKLIERWACEIADFFIKNKVGTVQMENLESMKRKEDSYFNIRLRGFWPYAEMQDKIEFKLKQYGIEIRKVAPNNTSKTCSRCGHLNNYFNFEYRRENKFPHFKCEKCNFKENADYNAALNISNPKLKSTKEEP

SEQ ID NO: 970 - protein, 726 aa, synthetic construct
SEVEFSHEYWMRHALTLAKRARDEREVPVGAILVLNNRVIGEGWNRAIGLHDPTAHAEIMALRQGGLVLQNYRLIDATLYVTFEPCVMCAGAMIHSRIGRVVFGVRNNKHGAAGSLVNVLNYPGMNHRVEITEGILADECAALLCDFYRMPRQVFNAQKKARSNINSGGSSGGSSGSETPGTSGSATPESSGGSSGGSAKNTITKTLKLRIVRPYNSAEVEKIVADEKNNREKVALEKNKNKVKEACSEHLKVAAYCTTQVERNACLFCKARKLDDKFYQKLRGQFPDAVFWQEISEIFRQLQKQAAEIYNQSLIELYYEIFIKGKGFANASRVEHYLSDVCYTRAAGLFKNAAIASGLRGKVKSNFRLKELRNMKSGLPTTKSDNFPIPLVRQKGGQYTGFEISNHDGDFIIKIPFGRWQAKKEIDRYRPWEKFDFEQVRKSPKPISLLLSTQRRKRNKGWSKDEGTEAEIEKVMNGDYQTSYIEVKRGSKTGEKSAWMLNLSIDVPKIDKGVDPRIIGGIDVGVKSPLVCAINDAFSRYSISDNDLFHFNKKMFARRRILLKKNGHKRAGHGAKNKLKPITIMTEKSKRFRKKLIERWACEIADFFIKNKVGTVQMENLESMKRKEDSYFNIRLRGFWPYAEMQNKIEFKLKQYGIVVRKVAPNNTSKTCSRCGHLNNYFNFEYRKRNKFPHFKCEKCNFKENADYNAALNISNPKLKSPKEEP

SEQ ID NO: 971 - protein, 726 aa, synthetic construct
SEVEFSHEYWMRHALTLAKRARDEREVPVGAVLVLNNRVIGEGWNRAIGLHDPTAHAEVMALRQGGLVMQNYRLIDATLYVTFEPCVMCAGAMIHSRIGRVVFGVRNSKRGAAGSLMNVLNYPGMNHCVEITEGILVDECAALLCDFYRMPRQVLNAQKKAQSSISPGGSSGGSSGSETPDASESVTPKSSGGSSGGSAKNTITKTLKLRIVRPYNSAEVEKIVADEKNNREKIALEKNKDKVKEACSEHLKVAAYCTTQVERSACLFCKARKLDDKFYQKLRGQFPDAVFWQEIGEIFRQLQKQAAEIYNQSLIELYYQIFIKGKGFANASSVEHYLSDVCYTRAAELFKNAAIASGLRSKIKSNFRLKELRNMKSGLPTTKSDNFPIPLVKQKGGQYTGFEISSHNDDFIIKIPFGRWQVKKEIDKYRPWEKFDFEQVRKSPKPISLLLSTQRRRRNKGWSKDEGTEAEIRKVMNGDYQTSYIEVKRGSKIGEKSAWMLNLSIDVPKVDKGVDPSIIGGIDVGVKSPLVCAINNAFSRYSISDNELFHFNKKMFARRRILLGKNRHKRAGHGVKNKLKPITILTEKSGRFRKKLIERWACEIADFFVKNKVGTVQMENLESMKRKEDSYFNIRLRGFWPYAEMQNKIEFKLKQYGIEIRKVAPNNTSKTCSKCGHLNNYFNFEYRKKNKFPHFKCERCNFKENADYNAALNISNPKLKSTKEEP

SEQ ID NO: 972 - protein, 726 aa, synthetic construct
NEVEFSHEYWMRRALTLAKRARDEREVPVGAVLVLNNRVIGEGWNRAIGLHDPTAHAEIMALRQGGLVMQNYRLTDATLYVTFEPCVMCAGAMIHGRIGRVVFGVRNSKRGAAGSLMNVLNYPGMNHCVEITEGILVDECAALLCDFYRMPRQVLNAQKKAQSSISSGGSSGGSSGGETPGASGSVTPKSSGGSSAGSTKDTITKTLKLRIVRPYNSAEVEKIVADEKNNREKIALEKNKDKVKEACSEHLKVAAYCTTQVERNACLFCKARKLDDRFYQKLRGQFPDAVFWQELGEILRQLQKQAAEIYNQSLIELYYEVFIKGKGIANASSVEHYLSDVCYTRAAELFKNAAIASGLRGKVKSNFRLKELKNMKSGLPTTKSDNFPIPLVKQKGGQYTGFEISSHNGDFIIKIPFGRWQVKKEIDKYRPWEKFDFEQVRKSPKPISLLLSTQRRKRNKGWSKDEGTEAEIRKVMSGDYQTSYIEVKRGSKTGEKSAWMLNLSIDVPKIDKGVDPSIIGGIDVGVKSPLVCAINNAFSRYSISDNDLFHFNKKMFARRRILLKKNGHKRAGHGAKNKLKPITIMTEKSKRFRRKLIERWACEIADFFIKNKVGTVQMENLESMKRKEDSYFNIRLRGFWPYAEMQNKIEFKLKQYGIEIRKVAPNNTSKTCSKCGHLNNYFNFEYRKKNKFPHFKCEKCNFKENADYNAALNISNPKLKSTKEEP

SEQ ID NO: 973 - protein, 726 aa, synthetic construct
SEVEFSHEYWMRHALTLAKRARDEREVPVGAVLVLNNRVIGEGWNRAIGLHDPTAHAEIMALRQGGLVMQNYRLSDATLYVTFEPCVMCAGAMIHSRIGRVVFGVRNSKRGAAGSLMNVLNYPGMNHCVEITEGILVDECAALLCDFYRMPRQVLSAQKKAQSSISSGGSSGGSSGSETPGARGSVTPKSSGGGSSGSAKNTITKTLQLRIVRPYNSAEVEKIVADEKNNREKIALEKNKDKVKEACSKHLKVASYCTTQVERNACPFCKARKLDDKFYQKLRGQFPNAVFWQELGEILRQLQKQAAEIYNQSLIELYYEIFIKGRGFANAGSVEHYLSDVCYTRAAELFKNAAIASGLRGKVKSNFRLKELKNMKSGLPTTKSDNFPIPLVKQKGGQYTGFEISSHDDDFIIKIPFGRWQVKKEIDKYRPWEKFDFEQVRKSPKPISLLLSTQRRKRNKGWSKDEGTEAEIRKVLNGDYQTSYIEVKRGSKTGEKSAWMLNLSINVPKIDKGVDPSIIGGIDVGVKSPLVCAINNAFSRYSISDNDLFRFNKKMFARRRILLKKNRHKRAGHGAKNKLKPISILTGKSERFRKKLIERWACEIADFFIKNKVGTVQMENLESMKRKEDSYFNIRLRGFWPYAEMQNKIEFKLKQYGIKIRKVAPNNTSKTCSMCGHLNNYFSFEYRKKNKFPHFKCEKCNFKENADYNAALNISNPKLMSTKEGP

SEQ ID NO: 974 - protein, 726 aa, synthetic construct
SEDEFSHEYWMRHALTLAKRARDGREVPVGAVLVLNNRIIGEGWNRAIGLHDPTAHAEIMALRQGGLVLQNYRLIDATLYVTFEPCVMCAGAMVHSRIGRVVFGVRNSKRGAAGSLMNVLDYPGMGHRVEITEGILADECAALLCDFYCMPRQVFNAQKRAQSSINSGGSSGGSSGSETPGTSESATPESSGGGSSGSAKNTITKTLQLRIVRPYNSAEVEKVVADEKNNREKIALEKNKDKVKEACSKHLKVASYCTTQVERNACPFCKARKLDDKFYQKLRGQFPDAVFWQELGEILRQLQKQAAEIYNQSLIELYYEIFIKGRGFANASSVEHYLSDVCYTRAAELFKNAAIASGLRGKVKSNFRLKELKNMKSGLPTTKSDNFPIPLVKQKGGQYTGFEISSHNDDFIIKIPFGRWQVKKEIDRYRPWEKFDFEQVRKSPKPISLLLSTQRRKRNKGWSKDEGTEAEIRKVMNGDYQTSYIEVKRGSKTGEKSAWMLNLSIDVPKIDKGVDPSIIGGIDVGVKSPLVCAINNAFSRYSISDNDLFRFNKKMFARRRILLKKNRHKRAGHGAKNKLKPISILTGKSERFRKKLIERWACEIADFFIKNKVGTVQMENLESMKRKEDSYFNIRLRGFWPYAEMQNKIEFKLKQYGIEIRKVAPNNTSRTCSKCGHLNNYFNFEYRRKNKFPHFKCEKCNFKEDADYNAALNISNPKLKSTKEEP

SEQ ID NO: 975 - protein, 726 aa, synthetic construct
SEVEFSHEYWMRHALTLAKRARDEREVPVGAVLVLNNRVIGEGWNRAIGLHDPTAHAEIMALRQGGLVMQNYRLIDATLYVTFEPCVMCAGAMIHSRIGRVVFGVRNSKHGAAGSLVNVLNYPGMNHRVEITEGILADECAALLCDFYRMPRQVFNAQKRAQSSINSGGSSGGSSGSETSGTSESATPESSGGSSDGSAKNTITKTLKLRIVRPYNSAEVEKIVADEKNNREKIALEKNKDKVKEACSKHLKVAAYCTTQVERNACLFCKARRLDDKFYQKLRGQFPDAVFWQEIGEIFRQLQKQAAEIYNQSLVELYYEILIKGKGIANASSVEHYLSDVCYTRAAKLFKNAAIASGLRNKIKSNFRLKELRNMKSGLPTTKSDNFPIPLVRQKGGQYAGFEISSHNDDFIIKIPFGRWQVKKEIDKYRPWEKFDFEQVRKSPKPISLLLSTQRRKRNKGWSKDEGTEAEIRKVMNGDYQTSYIEVKRGSKTGEKSTWMLNLSIDVPKIDKGVDPSIIGGIDVGVKSPLVCAINNAFSRYSISDNDLFRFNKKMFARRRILLKKNRHKRAGHGAKNKLKPISILTGKSERFRKKLIERWACEIADFFIKNKVGTVQMENLESMKGREDSYFNIRLRGFWPYAEMQSKIEFKLKQYGIKIRKVAPNNTSKTCSKCGHLNNYFNFEFRKKNKFPHFKCEKCNFKENADYNAALNISNPKLKSTKEEP

SEQ ID NO: 976 - protein, 726 aa, synthetic construct
SEVEFSHEYWMRRALTLAKRARDEREVPVGAVLVLNNRVIGEGWNRAIGLHDPTAHAEIMALRQGGLVTQNYRLIDATLYVTFEPCIMCAGAMIHSRIGRVVFGVRNSKRGAAGSLMNVLDYPGMNHRVEITEGILAGECAALLCDFYRMPRQVFNAQKKAQSNINPGGSSEGSSGSETPGTSESATPESSGGSSGGSAKNTITKTLKLRIVRPYNSAEVEKIVADEKNNREKIALEKNKDKVKEACSKHLKVASYCTTQVERNACLFCKARKLDDKFYQRLRGQFPDAVFWQELGEIFRQLQKQAAEIYNQSLIELYYEIFIKGKGLASASSVEHYLSDVCYTRAAELFKNAAIASGLRGKVKGNFRLKELKNMKSGLPTTKSDNFPIPLVKQKGGQYTGFEISSHNDDFIIKIPFGRWQVKKEIDKYRPWEKFDFEQVRKSPKPISLLLSTQRRKRNKGWSKDEGTEAEIRKVMNGDYQTSYIEVKRGSKTGEKSAWMLNLSIDVPRIDKGVDPSIIGGIDVGVKSPLVCAINNAFGRYSISDNDLFHFNKKMFARRRILLKKNRHKRAGHGAKNKLKPITILTEKSKRFRKKLIERWACEIADFFIKNKVGTVQMENLESMKRKEDSYFNIRLRGLWPYAEMQNKIEFKLKQYGIKIRKVAPNNTSKTCSKCGHLNNYFNFEYRKKNKFPHFKCEKCSFKENADYNAALNISNPKLKSTKEEP

SEQ ID NO: 977 - protein, 726 aa, synthetic construct
SEVEFSHEYWMRHALTLAKRARDEREVPVGAVLVLNNRVIGEGWNRTTGLHDPTAHAEIMALRQGGLVMQNHRLVDATLYVTFEPCVMCAGAMIHSRIGRVVFGVRNSKRGAAGSLTNVLNYPGMNHRVEITEGILVDECAALLCDFYRMPHQVFNARKKAQSSINPGGPSGGSSGSETPDTSESATPESSGGNSGGSAKNTITKTLKLRIVRPYNSAEVEKIVADEKNNRERIALEKNKDKVKEACSEHLKVAAYCTTQVNRNACLFCKARKLDDKFYQKLRGQFPDAVFWQELGEIFRQLQKQAAEIYNQSLIELYYEIFIKGKGFANASSVEHYLSDVCYTRAAELFKNAAIASGLRGKVRSNFRLKELKNMRSGLPTTKSDNFPIPLVKQKGGQYTGFEISSHHDDFIIKIPFGRWQVKKEINKYRPWEKFDFEQVRKSPKPISLLLSTQRRRRNKGWSKDEGTEAEIRKVMNGDYQISYIEVKRGSKIGEKGAWMLNLSIDVPKIDKGVDPSIIGGIDVGVKSPLVCAINNALSRYSISDNDLFHFNKKMFARRRILLKKNRHKRAGHGARNKLKPITVLTEKSERFRKKLIERWACEIAYFFIKNKVGTVQMENLESMKRREDSYFNTRLRGFWPYAEMQNKIEFKLKQYGIEVRKVAPNNTSKTCSKCGHLNNYFNFEYRKKNKFPHFKCEKCNFKENADYNAALNISNPRLKSTKEEP

SEQ ID NO: 978 - protein, 726 aa, synthetic construct
SEVEFSHEYWMRHALTLAKRARDEREVPVGAVLVLNNRVIGEGWNRAIGLHDPTAHAEIMALRQGGLVMQNYRLIDATLYVTFEPCVMCAGAMIHSRIGRVVFGVRNSKRGAAGSLMNVLNYPGMNHRVEITEGILAGECAALLCDFYRMPRQVLNAQKKARSCINSGGSSGGSSGSETPGTSERATPETPGGSSGGSAKNTITKTLKLRIVRPYNSAEVEKIVADEKDNRERIALEKNKGKVKEACSKHLKVAAYCTTQVERNACLFCKARKLDDKFYQKLRGQFPDAVFWQEIGGIFRQLQKQAAEIYNQSLIELYYEIFIKGKGIANASSVEHYLSDVCYTRAAELFKNAAIASGLRNKVKSNFRLKELKSMKSGLPTTKSDNFPIPLVRQKGGQYTGFEISNHNSDFIIKIPFGRWQAKKEIDKYRPWEKFNFEQVRKSPKPISLLLSTQRRKRNKGWSKDEGTEAEIKKVMNGDYRTSYIEVKRGSKIGEKSAWMLNLSIDVPKIDKGVDPSIIGGIDVGVKSPLVCAINNAFSRYSISDNDLFRFNKKMFARRRILLEKNRHKRAGHGVKNKLKPITILTEKSRRFRKKLIERWACEIANFFIKNRVGTVQMENLESMKRKEDSYFNIRLRGFWPYAEMQNKIEFKLKQYGIKIRKVAPNNTSKTCSKCGHLNNYFNFEFRKKNKFPHFKCEKCNFKEDADYNAALNISNPKLKSTKEEP

SEQ ID NO: 979 - protein, 726 aa, synthetic construct
SEVEFSHEYWMRHALTLAKRARDEREVPVGAVLVLNNRVIGEGWNRAIGLHDPTAHAEIMALRQGGLAMQNYRLVDATLYVTFEPCVLCAGAMVHSRIGRVVFGARNSKRGAAGSLMNILNYPGMNHRVEITEGILADECAALLCDFYCMPRQVFNAQKKAQSSINSGGSSGGSSGSETPGTSESATPESSGGSSGGSAKNTITKTLKLRIVRPYNSAEVERIVADEKDNRERIALEKNKGKVKEACSKHQKVAAYCTTQVERNACLFCKARKLDDKFYQKLRGQFPDAVFWQEIGEIFRQLQKQAAEIYNQSLIELYYEIFIKGKGFANASSVEHYLSDVCYTRAAELFKNAAIASGLRGKVKSNFRLKELKNMKSGLPTTKSDNFPIPLVRQKGGQYTGFEISNHNGDFIIKIPFGRWQVKKEIDKYRPWEKFDFEQVRKSPKPISLLLSTQRRKRNKGWSKDEGTEAEIRKVMNGDYQTSYIEVKRGSKIGEKSAWMLNLSIDVPKIDKGVDPSTIGGIDVGVKSPLVCAINNAFSRYSISDNDLFRFNKKMFARRRILLRKNRHKRAGHGAKNKLKPITILTGKSERFRKKLIERWACEIADFFIKNKVGTVQMENLESMKRKEDSYFNIRLRGFWPYAEMQNKIEFKLKQYGIKIRKVAPNNTSKTCSKCGHLNNYFNFEYRKKNKFPHFKCEKCNFKENADYNAALNISNPKLKSTKEKP

SEQ ID NO: 980 - protein, 726 aa, synthetic construct
SEVEFSHEYWMRRALTLAKRARDEREVPVGAVLVLNNRVIGEGWNRAAGLHDPTAHAEIMALRQGGLVMQNYRLIEATLYVTFEPCIMCAGAMIHSRIGRVVFGVRNSKRGAAGSLMNVLNYPGMSHRVEITEGILADECAALLCDYYRMPRQVFNARKKAQSSINSGGSSDGGSGSETPGTSESATPESSGGSSGGSAKNTITKTLKLRIVRPYNSAEVEKIVADEKNNREKIALEKNKDKVKEACSKHLKVAAYCTTQVERNACLFCKARKLDDKFYQKLRGQFPDAVFWQELGEILRQLQKQAAEIYNQSLIELYYEIFIKGRGLANASSVEHYLSDVCYTRAAELFKNAAIASGLRGKVKSNFRLKELKNMKSGLPTTKSDNFPIPLVKQKGGQYTGFEISSHNDDFIIKIPFGRWQVKKEIDKYRPWEKFDFEQVRKSPKPISLLLSTQRRKRNKGWSKDEGTEAEIKKVMNGDYQISYIEVKRGNKIGEKSAWMLSLSVDVPKIDKGVDPSIIGGIDVGVKSPLVCAINNALSRYSISDNDLFHFNKKVFARRRILLKKNRHKRAGHGAKNKLKPITILTEKSERFRKKLIERWACEIANFFIKNKVGTVQMEDLESMKRKEDSYFNVRLRGFWPYAEMQNKIEFKLKQYGIEIRKVAPNNTSKTCSKCGHPNNYFNFEYRKKNKFPHFKCEKCNFKEDADYNAALNISNPKQKSAKEEP

SEQ ID NO: 981 - protein, 726 aa, synthetic construct
SEVEFSHEYWMRHALTLAKRARDEREVPVGAILVLNNRVIGEGWNRAIGLHDPTAHAEIMALRQGGLVMQNYRLIDATLYVTFEPCVMCAGAMIHSRIGRVVFGVRNSKHGAAGSLVNVLNYPGMNHRVEITEGILADECAALLCDFYRMPRQVFNARKKAQSSINPSGSSGGSSGSATPGTSESATPESSGGGFGSSAKNTITKTLQLRIVRPYNSAEVEKIVADEKNNREKIALEKNKDKVKEACSKHLKVASYCTTQVERNACLFCKARKLDDKFYQKLRGQFPDAVFWQELGEILRQLQKQAAEIYNQSLIELYYEIFIKGKGFANASSVEHYLSDVCYTRAAELFKNAAIASGLRGKVKSNFRLKELKNMKSGLPTTKSDNFPIPLVKQKGGQYTGFEISSHNDDFIIKIPFGRWQVKKEIDKYRPWEKFDFEQVRKSPKPISLLLSTQRRKRNKGWSKDEGTEAEIRKVMNGDYQTSYIEVKRGSKIGEKSAWMLNLSIDVPKIDKGVDPSIIGGIDVGVKSPLVCAINNAFSRYSISDNDLFHFNKKVFARRRILLKKNRHRRAGHGAKNKLKPITILTEKSKRFRKKLIERWACEITDFFIKNKVGTVQMENLESMKRKEDSYFNIRLRGFWPYAEMQNKIEFKLKQYGIEIRKVAPNNTSRTCSKCGHLNNYFNFEYRRKNKFPLFKCEKCNFKEDADYNAALNISNPKLKSTKEEP

SEQ ID NO: 982 - protein, 726 aa, synthetic construct
SEVEFSHEYWMRHALSLAKRARDEREVPVGAVLVLNNRIIGEGWNRAVGLHDPTAHAEIMALRQGGLVMQNYRLTDATLYVTFEPCVMCAGAMVHSRIGRVVFGVRNSKRGAAGSLMNVLNYPGVNHCVEITEGILVDECAALLCDFYRMPRRVLNAQKKAQSSISSGGSSGGSGGGETPGASESVTPKSSGGSSAGSTKNTITKTLQLRIVRPYNSAEVEKIVTDEKNNREKIALEKNKDKVKEACSKHLKMASYCTTQVERNACLFCKARKLDDKFYQKLRGQFPDAVFWQELGGIFRQLQKQAAEIYNQSLIELYYEIFIKGKGIANASSVEHYLSDVCYTRAAELFKNAAIASGLRNKIKSNFRLKELRNMKSGLPTTKSDNFPIPLVRQKGGQYTGFEISNHDGDFIIKIPFGRWQVKKEINKHRPWEKFDFEQVRKSPKPISLLLSTQRRKRNKGWSKDEGTEAEIRKVMNGDYQTSYIEVKRGSKIGEKSAWMLNLSIDVPKIDKGVDPSIVGGIDVGVKSPLVCAINNAFSRYGISDNDLFRFNKKMFARRRILLGKNRHKRAGHGVKNKLKPITILTEKSGRFRKKLIERWACEIADFFVKNKVGTVQMENLESLKRKEDSYFNIRLRGFWPYAEMQNKIEFKLKQYGIKVRKVAPNNTSKTCSKCGHLNNYFSFEYRKKNKFPHFKCEKCNFKENADYNAALNISNPKLKSTKGEP

SEQ ID NO: 983 - protein, 726 aa, synthetic construct
SEVEFSHEYWMRHALTLAKRARDEREVPVGAVLVLNNRVIGEGWNRAIGLHDPTAHAEIMALRQGGLVMQNYRLIDATLYVTFEPCVMCAGAMVHSRIGRVVFGVRNGKRGAAGSLMNVLDYPGMGHRVEITEGILADECAALLCDFYCMPRQVFNAQKRAQSSINSGGSSGGSSGSETPGTSESATPESSGGGSSGSAKSTITKTLQLRIVRPYNSAEVEKIVADEKNNREKIALEKNKDKVKEACSKHLKVASYCTTQVGRNACPFCKARKLDDKFYQKLRGQFPDAVFWQEIGEIFRQLQKQAAEVYNQSLVELYYEILIEGKGIANASSVEHYLSDVCYTRAAELFKNAAIASGLRNKIKSNFRLKELRNMKSGLPTTKSDNFPIPLVRQKGGQYTGFEISNHDGDFIIKIPFGRWQVKKEIDKYRPWEKFDFEQVRKSPKPISLLLSTQRRKRNKGWSKDEGTEAEIRKVMNGDYQTSYIEVKRGSKIGEKSAWMLNLSIDVPKIDKGVDPSIIGGIDVGVKSPLVCAINNAFSRYSISDNDLFHFNKKMFARRRILLKKNRHKRAGHGAKNKLKPISILTEKSKRFRKKLIERWACEIADFFIKNKVGTVQMENLESMKRKEDSYFNIRLRGFWPYAEMQNKIEFKLKQYGIEIRKVAPNNTSKTCSKCGHLNNYFNFEYRKMNKFPHFKCEKCNFKENADYNAALNISNPKLKSTKEEP

SEQ ID NO: 984 - protein, 726 aa, synthetic construct
SEVEFSHEYWMRHALTLAKRARDGREVPVGAVLVLNNRVIGEGWNRAIGLHDPTAHAEIMALRQGGLVMQNYRLIDATLYVTFEPCVMCAGAMVHSRIGRVVFGVRNSKRGAAGSLMNVLDYPGMGHRVEITEGILADECAALLCDFYCMPRQVFNAQKRAQSSINSGGSSGGGSGSETPGASESVTPKSSGGSSGGSAKNTITKTLKLRIVRPYNSAEVEKIVADEKNNREKIALEKNKGKVKEACSKHLEVAAYCTTQVERNACLFCKARKLDDKFYQKLRGQFPDAVFWQEISEIFRQLQKQAAEVYNQSLIELYYEIFIKGKGFANASSVEHYLSDVCYTRAAELFKNAAIASGLRGKVKSNFRLKELKNMKSGLPTTKSDNFPIPLVKQKGGQYTGFEISSHNDDFIIKIPFGRWQVKEEIDKYRPWEKFDFEQVRRNPKPISLLLSTQRRKRNKGWSKDEGTEAEIRKVMNGDYQTSYIEVKRGSKIGEKSAWMLNLSIDVPKVDKGVDPSIIGGIDVGVKSPLVCAINDAFSRYSISDNDLFRFNKKMFARRRILLKKNRHKRAGHGAKNKLKPISILTEKSKRFRKKLIERWACEIADFFIKNKVGTVQMENLESMKRKEDSYFNIRLRGFWPYAEMQNKIEFKLKQYGIEIRKVAPNNTSKTCSKCGHLNNYFNFEYRKKNKFPHFKCEKCNFKENADYNAALNISNPKLKSTKEEP

SEQ ID NO: 985 - protein, 726 aa, synthetic construct
SEVEFSHEYWMRHALTLAKRARDEREVPVGAILVLNNRVIGEGWNRAISQHDPTAHAEIMALRQGGLVMQNHRLIDATLYVTFEPCVMCAGAMIHSRIGRVVFGVRNSKHGAAGSLVNVLNYPGMNHRVEITEGILAGECAALLCDFYRMPRQVFNAQKKAQSTINSGGSSGGSSSSETPGTSGSATPEGSGGSSGGSAKNTVTKTLKLRIVRPYNSAEVEKIVADEKNNREKIALEKNKDKVKEACSKHLKVASYCTTQVERNACLFCKARKLDDKFYQKLRGQFPDAVFWQELGEIFRQLQKQAAEIYNQSLIELYYEIFIKGKGFANASSVEHYLSDVCYTRAAEMFKNAAIASGLRGKVKSNFRLKELKNMKSGLPTTKSDNFPIPLVKQKGGQYTGFEISSHNDDFIIKIPFGRWQVKKEIDKYRPWEKFDFEQVRKSPKPISLLLSTQRRKRNKGWSKDEGTEAEIRKVMNGDYQISYIEVKRGSKIGEKSTWMLNLSIDVPKIDKGVDPSIIGGIDVGVKSPLVCAINNAFGRYSISDNDLFRFNKKMFARRRILLKKNRHKRAGHGAKNKLKPISILTGKSERFRKKLIERWACEIADFFIKNKVGTVQMENLESMKRKEDSYFNIRLRGFWPYAEMQNKIEFKLKQYGIEIRKVAPNNTSKTCSKCGHLNNYFNFEYRKKNKFPHFKCEKCNFKENADYNAALNISNPKLKSTKEKP

SEQ ID NO: 986 - protein, 726 aa, synthetic construct
SEVEFSHEYWMRHALTLAKRARDEREVPVGAILVLNNRVIGEGWNRAIGLHDPTAHAEIMALRQGGLVMQNYRLIDATLYVTFEPCVMCAGAMIHSRIGRVVFGVRNSKRGAAGSLTNVLNYPGMNHRVEITEGILVDECAALLCDFYRMPRQVFNAQKKAQSTINSGGSSGGSSGSETPGTSESPTPESSGGSPGGSAKNTVTKTLKLRIVRPYNSTEVEKIVADEKNNREKIALEKNKDKVKEACSKHLKVAAYCTTQVERNACLFCKARKLDDKFYQKLRGQFPDAVFWQEVGEIFRQLQKQAAEIYNQSLIELYYEIFIKGKGFANASSVEHYLSDVCYSRAAELFKNAAIASGLRGKVKSNFRLKELKNMKSGLPTTKSDNFPIPLVKQKGGQYTGFEISSHNDDFIIKIPFGRWQAKKEIDKYRPWEKFDFEQVRKSPKPISLLLSTQRRKRNRGWSKDEGTEAEIRKVMNGDYQTSYIEVKRGSKIGEKSAWMLSLSIDVPKIDKGVDPSIIGGIDVGVKSPLVCAINNAFSRYSISDNDLFRFNKKMFARRRILLGKNRHKRAGHGVKNKLKPITILTEKSGRFRKKLIERWACEIADFFVKNKVGTVQMENLESMKRKEDSYFNIRLRGFWPYAEMQNKIEFKLKQYGIKVRKVAPNNTSKTCSKCGHLNNHFSFEYRKKNKFPHFKCEKCNFKENADYNAALNISNPKLKSTKEEP

SEQ ID NO: 987 - protein, 726 aa, synthetic construct
SEVEFSHEYWMRHALTLAKRARDEREVPVGAVLVLNNRVIGEGWNRAIGLHDPTAHAEIMALRQGGLVMQNYRLIDATLYVTFEPCVMCAGAMIHSRIGRVVFGVRNSKHGAAGSLVNVLNYPGMNHRVEITEGILADECAALLCDFYRMPRQVFGARRKAQSSINPGGSSGGSSSSETPGTSESPTPESPGGSSGGSAKNTITKTLKLRIVRPYNSAEVEKIVADEKNNREKIALEKNKDKVKEACSKHLKMASYCTTQVERNACLFCKARKLDDKFYQKLRGQFPDAVFWQEIGEIFRQLQKQAAEIYNQSLVELYFEIFIKGKGFANASSVEHYLSDVCYTRAAELFKNAAIASGLRGKVKSNFRLKELKNMKSGLPTTKSDNFPIPLVKQKGGQYTGFEISSHDDDFIIKIPFGRWQVKKEIDKYRPWEKFDFERVRKSPKPISLLLSTQRRKRNKGWSKDEGTEAEVRKVMNGDYRTSYIEVKRGSKTGEKSAWMLNLSIDVPKIDKGVDPSIIGGIDVGVKSPLVCAINNAFSRYSISDNDLFRFNKKMFARRRILLKKNRHKRAGHGAKNKLKPISILTEKSKRFRKKLIERWACEIADFFIKNKVGTVQMENLESMKRKEDGYFNIRLRGFWPYAEMQNKIEFKLKQYGIEIRKVAPNNTSKTCSKCGHLNNYFNFEYRKTNKFPHFKCEKCNFKEDADYNAALNISNPKLKSTKEEP

SEQ ID NO: 988 - protein, 726 aa, synthetic construct
SEVEFSHEYWMRHALSLAKRARDEREVPVGAVLVLNNRIIGVGWNRAIGLHDPTAHAEIMALRQGGLVMQNHRLVDATLYVTFEPCVMCAGAMIHSRIGRVVFGVRNSKRGAAGSLTNVLNYPGMNHRVEITEGILVDECAALLCDFYRMPRQVFNAQKKAQSTTNSGGSSGGSSGSETPGTSESPTPESSGGSPGGSAKNTITKTLKLRIVRPYNSAEVEKIVADEKNNREKIALEKNKDKVKEACSKHLKVAAYCTTQVERNACLFCKARKLDDKFYQKLRGQFPDAVFWQEIGEIFRQLQKQAAEIYNQSLIELYYEIFIKGRGFANASSVEHYLSDVCYTRAAELFKNAAIASGLRGKVKSNFRLKELKNMKSGLPTTKSDNFPIPLVKQKGGQYTGFEISSHNDDFIIKIPFGRWQVKKEIDKYRPWEKFDFEQVRKSPKPISLLLSTQRRKRNKGWSKDEGTEAEIRKVMNGDYQTSYIEVKRGSKTGEKSAWMLNLSIDVPKIDKGVDPSIIGGIDVGVKSPLVCAINNAFSRYSIGDNDLFHFNKKMFARRRILLKKNRRKRAGHGAKNKLKPITILTEKSKRFRKKLIERWACEIADFFIRNKVGTVQMENLESMKRKEDSYFNIRLRGFWPYAEMQNKIEFKLKQYGIEIRKVAPNNTSRTCSKCGHLNNYFNFEYRKKNKFPHFKCEKCNFKENADYNAALNISNPKLKSTKEEP

SEQ ID NO: 989 - protein, 726 aa, synthetic construct
SEVEFSHEYWMRHALTLAKRARDEREVPVGAVLVLNNRVIGEGWNRTTGLHDPTAHAEIMALRQGGLVTQNHRLVDATLYVTFEPCVMCAGAMIHSRIGRVVFGVRNSKRGAAGSLTNVLNYPGMNHRVEITEGILVDECAALLCDFYRMPRQVFNAQKKAQSTINSGGSSGGSSGSETPGTSESPTPESSGGSPGGSAKNTITKTLKLRIVRPYNSAEVEKIVADEKNNREKIALERNKDKVKEACSKHLKVAAYCTTQVERNACLFCKARKLDDKFYQKLRGQFPDAVFWQEIGEIFRQLQKQAAEIYNRSLIELYYEIFIKGKGIANASRVEHYLSDVCYTRAAELFKNAAIASGLRNRIKSNFRLKELKNMKSGLPTTKSDNFPIPLVKQKGGQYTGFEISSHNDDFIIKIPFGRWQVKKEIDRYRPWEKFDFEQVRKSPKPISLLLSTQRRKRNKGWSKDEGTEAEIRKVMNGDYQTSYIEVKRGSKIGEKSAWMLSLSIDVPKIDKGVDPSTIGGIDVGVKSPLVCAINNAFCRYSISDNDLFHFNKKMFARRRILLKKSRHKRAGHGAKNKLKPISILTEKSKRFRKKLIERWACEIADFFIKNKVGTVQMENLESMKRKEDSYFNIRLRGFWPYAEMQNKIEFKLKQYGIKVRKVAPNNTSKTCSKCGHLNNYFSFEYRKKNKFPHFKCEKCNFKENADYNAALNISNPKLKSTKEEP

SEQ ID NO: 990 - protein, 726 aa, synthetic construct
SEVEFSHEYWMRHALTLAKRARDEREVPVGAVLVLNNRVIGEGWNRAIGLHDPTAHAEIMALRQGGLVMQNYRLIDATLYVTFEPCVMCAGAMIHSRIGRVVFGVRNSKHGAAGSLVNVLNYPGMNHRVEITEGILADECAALLCDFYRMPRQVFNAQKKARSNINSGGSSGGSSGSETPGTSESPTPESSGGSFGGSAKNTITKTLKLRIVRPYNSAEVEKIVADEKNNREKIALEKNKDKVREACSEHLKVAAYCTTQVERSACLFCKARKLDDKFYQKLRGQFPDAVFWQETGEIFRQLQRQAAEIYNQSLIELYYEIFIKGKGFANASSVEHYLSDVCYTRAAELFKNAAIASGLRGKVKSNFRLKELKNMKSGLPTTKSDNFPIPLVKQKGGQYTGFEISSHNDDFIIKIPFGRWQVKKEIDKYRPWEKFDFEQVRKSPKPISLLLSTQRRKRNKGWSKDEGTEAEIRKVMNGDYQTSYIEVKRGSKIGEKSAWMLNLSIDVPKIDKGVDPSIIGGIDVGVKSPLVCAINNAFSRYSISDNDLFRFNKKMFARRRILLKKNRHKRAGHGAKNKLKPTSILTEKSRRFRKKLIERWACEIADFFIKNKVGTVQMENLESMKRREDSYFNIRLRGFWPYAEMQNKIEFKLKQYGIEIRKVAPNNTSKTCSKCGHLNNHFNFEYRRRNKFPHFKCEKCNFKENADYNAALNISNPKLKGTKEGP

SEQ ID NO: 991 - protein, 726 aa, synthetic construct
SEVEFSHEYWMRHALTLAKRARDEREVPVGAVLVLNNRVIGEGWNRTTGLHDPTAHAEIMALRQGGLVMQNHRLVDATLYVTFEPCVMCAGAMIHSRIGRVVFGVRNSKRGAAGSLTNVLNYPGMNHRVEITEGILVDECAALLCDFYRMPRQVFNAQKRAQSTINTGGSSGGSSGSETPGTSESPTPESSGGSSGGSAKNTITKTLKLRIVRPYNSAEVEKIVADEKNNRERIALEKNKDKVKEACSKHLKVAAYCTTQVERNACLFCKARKLDDKFYRELRGQFPDAVFWQEIGEIFRQLQKQAAEIYNQSLIELYYEIFIKGKGFANASSVEHYLSDVCYTRAAELFKNAAIASGLRGKVKSNFRLKELKNMKSGLPTTKSDNFPIPLVKQKGGQYTGFEISSHNDDFIIKIPFGRWQVKKEIDKYRPWEKFDFEQVRKSPKPISLLLSTQRRKRNKGWSKDEGTEAEIRKVMNGDYRTSYIEVKRGSKTGEKSAWVLNLSIDVPKIDKGVDPSIIGGIDVGVKSPLVCAINNAFSRYSISDNDLFRFNKKMFARRRILLKKNRHKRAGHGARNKLKPITVLTEKSERFRKKLIERWACEIANFFIKNKVGTVQMENLESMKRREDSYFNIRLRGFWPYAEMQSKIEFKLKQYGIKIRKVAPNNTSKTCSKCGHLNNYFNFEFRKKNKFPHFKCEKCNFKEDADYNASLNISNPKLKSTKEEP

SEQ ID NO: 992 - protein, 726 aa, synthetic construct
SEDEFSHEYWMRHALTLAKRARDGREVPVGAVLVLNNRVIGEGWNRAIGLHDPTAHAEIMALRQGGLVMQNYRLTDATLYVTFEPCVMCAGAMVHSRIGRVVFGVRNSKRGAAGSLMNVLNYPGMNHCVEITEGILVDECAALLCDFYRMPRQVLNAQKKAQSSISPGGSSGGSSGSETPGASESVTPKSSGGSSAGSTKNTITKTLKLRIVRPYNSAEVEKIVADEKNSREKIALEKNKDKVKEACSEHLKVAAYCTTQVERNACLFCKARKLDDRFYQKLRGQFPDAVFWQEIGEIFRQLQKQAAEIYNQSLIELYYEIFIKGKGFANASSVEHYLSDVCYTRAAELFKNAAIASGLRGKVKSNFRLKELKNMKSGLPTTKSDNFPIPLVKQKGGQYTGFEISSHNDDFIIKIPFGRWQVKEEIDKYRPWEKFDFEQVRKNPKPISLLLSTQRRKRNKGWSKDEGTEAEIRKVMNGDYQTSYIEVKRGSKIGEKSAWMLNLSIDVPKIDKGVDPSIIGGIDVGVKSPLVCAINNAFSRYSIGDNDLFRFNKKMFARRRILLGKNRHKRAGHGVKNKLKPITILTEKSGRFRKKLIERWACEIADFFVKNKVGTVQMENLESMKRKEDSYFNIRLRGFWPYAEMQNKIEFKLKQYGIRVRKVAPNNTSKTCSKCGHLNNYFSFEYRKKNKFPHFKCEKCNFKENADYNAALNISNPKLKSTKEEP

SEQ ID NO: 993 - protein, 726 aa, synthetic construct
SEVEFSHEYWMRHALTLAKRARDEREVPVGAVLVLNNRIIGEGWNRAIGLHDPTAHAEIMALRQGGLVMQNHRLVDATLYVTFEPCVLCAGAMVHSRIGRVVFGVRNSKRGAAGSLMNVLNYPGMNHRVEITEGILADECAALLCDFYRMPRQVFNARKKAQSSINPSGSSGGSSGSVTPGTSESATPESSGGGFGGSAKNTITKTLQLRIVRPYNSAEVEKIMADEKNNREKIALEKNKDKVKEACSKHLKVASYCTTQVERNACLFCKARKLDDKFYQKLRGQFPDAVFWQELGEIFRQLQKQAAEIYNQSLIELYYEIFIKGRGFANTSSVEHYLSDVCYTRAAELFKNAAIASGLRGKVKSNFRLKELKNMKSGLPTTKSDNFPIPLVKQKGGQYTGFEISSHDDDFIIKIPFGRWQVKKEIDKFRPWEKFDFEQVRKSPKPISLLLSTQRRKRNKGWSRDEGTEAEIRKVMNGDYQTSYIEVKRGSKIGEKSAWMLNLSIDVPKIDKGVDPSIIGGIDVGVKSPLVCAINNALSRYSISDNDLFHFNKKMFARRRILLRKNRHKRAGHGAKNKLKPITIMTEKSKRFRKKLIERWACEIADFFIKNKVGTVQMENLESMKKKEDSYFNIRLRGFWPYAEMQNKIEFKLKQYGIVVRKVAPNNTSKTCSKCGHLNNYFNFEYRKKNKFPHFKCEKCNFKEDADYNAALNISNPKLKSTRGEP

SEQ ID NO: 994 - protein, 726 aa, synthetic construct
SEVEFSHEYWMRHALTLAKRARDEREVPVGAVLVLNNRVIGEGWNRAIGLHDPTAHAEIMALRQGGLVMQNYRLVDATLYVTFEPCVLCAGAMVHSRIGRVVFGVRNSKRGAAGSLMNVLNYPGMNHRVEITEGILADECAALLCDFYRMPRQVFNAQKKARSNINSGGSSGGSSGSETPGTSESATPESSGGSSGGSAKNTITKTLKLRIVRPYNSAEVERIVADEKDNREKVALEKNKDKVKEACSEHLKVAAYCTTQVVRNACLFCKARKLDDKFYQKLRGRFPDAVFWQEIGEIFRQLQKQAAEIYNQSLIELYYEIFIKGKGFANASSVEHYLSDVCYTRAAELFKNAAIASGLRGKVKSNFRLKELKNMKSGLPTTKGDNFPIPLVKQKGGQYTGFEISSHNDDFIIKIPFGRWQVKKEIDKYRPWEKFDFEQVRKSPKPISLLLSTQRRKRNKGWSKDEGTEAEIRKVMNGDYQTSYIEVKRGSKTGEKSAWMLNLSIDVPKIDKGVNPSIIGGIDVGVKSPLVCAINNAFSRYSISDNDLFHFNKKMFARRRILLKKNGHKRAGHGAKNKLKPITIMTEKSKRFRKKLIERWACEIADFFIKNKVGTVQMENLESMKRKEDSYFNIRLRGFWPYAEMQNKIEFKLKQYGIVVRKVAPNNTSKTCSKCGHLNNYFNFEYRKKNKFPHFKCEKCNFKEDADYNAALNISNPKLKSTKGEP

SEQ ID NO: 995 - protein, 726 aa, synthetic construct
SEVEFSHEYWMRHALTLAKRARDEREVPVGAVLVLNNRVIGEGWNRAIGLHDPTAHAEIMALRQGGLVMQNYRLIDATLYVTFEPCVMCAGAMVHSRIGRVVFGVRNSKRGAAGSLMNVLDYPGMGHRVEITEGILADECAALLCDFYRMPRQVFNTRKKAQSSINPSGSSGGSSGSVTPGTSESATPESSGGSSAGSTKNTITKTLKLRIVRPYNSAEVEKIVADEKNNREKIALEKNKDKVKEACSKHLKVAAYCTTQVERNACLFCKARRLDDKFYQKLRGQFPDAVFWQEIGEIFRQLQKQAAEVYNQSLVELYYEILIKGKGIANASSVEHYLSDVCYTRAAELFKNAAIASGLRNKIKSNFRLKELRNMKSGLPTTKSDNFPIPLVRQKGGQYTGFEISNYNGDFIIKIPFGRWQVKKEINKHRPWEKFDFEQVRKSPKPISLLLSTQRRKRNKGWSKDEGTEAEIRKAMNGDYQTSYIEVKRGSKIGEKSAWMLSLSIDVPKIDKGVDPRIIGGIDVGVKSPLVCAINNVLSRYSISDNDLFHFNKKMFARRRILLKKNGHKRAGHGAKNKLKPITIMTEKSKRFRKKLIERWACEIADFFIKNKVGTVQMENLESMKRKEDSYFNIRLRGFWPYAEMQNKIEFKLKQYGIEIRKVAPNNTSKTCSKCGHLNNYFNFEYRKRNKFPHFKCEKCNYKEDADYNAALNISNPKLKSTKEEP

SEQ ID NO: 996 - protein, 726 aa, synthetic construct
SEVEFSHEYWMRHALTLAKRARDEREVPVGAVLVLNNRVIGEGWNRAIGLHDPTAHAEIMALRQGGLVMQNYRLVDATLYVTFEPCVLCAGAMVHSRIGRVVFGVRNSKRGAAGSLLNVLNYPGMNHRVEITEGILADECAALLCDFYRMPRQVFSAQKKAQSSINSGGSSGGSSGSKTPGTSESATPESSGGGSSGSAKNTITKTLQLRIVRPYNSAEVEKIVADEKNNREKIALEKNKDKVKEACSKHLKVASYCTTQVERNACPFCKARKLDDKFYQKLRGQFPDAVFWQELGEILRQLQRQAAEIYNQSLIELYYEIFIKGRGFANASSVEHYLSDVCYTRAAELFKNAAIASGLRGKVKSNFRLKELKNMKSGLPTTKSDNFPIPLVKQKGGQYTGFEISSHNDDFIIKIPFGRWQVKKEIDKYRPWEKFDFEQVRKSPKPISLLLSTQRRKRNKGWSKDEGTEAEIRKVMNGDYQTSYIEVKRGSKTGEKSAWMLNLSIDVPKIDKGVDPSIIGGIDVGVKSPLVCAINNAFSRYSISDNDLFRFNKKMFARRRILLKKNRHKRAGHGAKNKLKPISILTGKSERFRKKLIERWACEIADFFIKNKVGTVQMENLESMKRKEDSYFNIRLRGFWPYAEMQNKIEFKLKQYGIKVRKVAPNNTSKTCSKCGHLNNYFNFEYRKMSKFPHFKCEKCNFKENADYNAALNISNPKLKSTKEEP

SEQ ID NO: 997 - protein, 726 aa, synthetic construct
SEVEFSHEYWMRHALTLAKRARDEREVPVGAILVLNNRVIGEGWNRAIGLHDPTAHAEIMALRQGGLAMQNYRLTDATLYATFEPCVMCAGAMIHSRIGRVVFGVRNSKHGAAGSLMNVLNYPGMNHRVEITEGILADECAGLLCDFYRMPRQVFSARKKAQSSINPGGSSGGSSGGKAPGTSESATLESSGGSSGSSAKNTITKTLKLRIVRPYNSAEVEKIVADEKNNREKIALEKNKDKVKEACSEHLKVAAYCTTQVERNACLFCKARKLDDKFYQKLRGQFPDAVFWQEIGEIFRQLQRQAAEIYNQSLIELYYEIFIKGKGFANASSVEHYLSDVCYARAAELFKNAAIASGLRGKVKSNFRLKELKNMKSGLPTTKSDNFPIPLVKQKGGQYTGFEISSHNDDFIIKIPFGRWRVKKEIDKYRPWEKFDFEQVRKSPKPISLLLSTQRRKRNKGWGKDESTEAEIRKVMNGDYQTSYIEVKRGSKIGEKSAWMLNLSIDVPKIDKGVNPSIIGGIDVGVKSPLVCAINNALSRYSISDNDLFHFNKKMFARRRILLRKNRHKRAGHGAKNKLKPITMMTEKSKRFRKKLIERWACEIADFFIKNKVGTVQMENLESMKRKEDSYFNIRLRGFWPYAEMQNKIEFKLKQYGIVVRKVAPNNTSKTCSKCGHLNNYFNFEYRKKNKFPHFKCEKCNFKEDADYNAALNISNPKLKSSKGEP

SEQ ID NO: 998 - protein, 726 aa, synthetic construct
SEVEFSHEYWMRHALTLAKRARDEREVPVGAVLVLNNRAIGEGWNRAIGLHDPTAHAEIMALRQGGLVMQNYRLTDATLYVTFEPCVMCAGAMIHSRIGRVVFGVRNSKRGAAGSLMNVLNYPGMNHCVEITEGILVDECAALLCDFYRMPRQVLNAQKKAQSSISSGGSSGGSSGSETPGASGSVTPKSSGGSSAGSTKDTITKTLKLRIVRPYNSAEVEKVVADEKNNREKIAIEKNKDMVKEACSKHLKVASYCTTQVERNACLFCKARKLDDKFYQKLRGQFPDAVFWQELGEIFRQLQKQAAEIYNQSLIELYYEIFIKGKGFANASSVEHYLSDVCYTRAAELFKNAAIASGLRGKVKSNFRLKELKNMKSGLPTTKSDNFPIPLVKQKGGQYTGFEISSHNDDFIIKIPFGRWQVKKEIDKYRPWEKFDFEQVRKSPKPISLLLSTQRRKRNKGWSKDEGTEAEIRKVMNGDYQTSYIEVKRGSKIGEKSAWMLNLSIDVPKIDKGVDPSIIGGIDVGVKSPLVCAVNNAFSRYSISDNELFHFNKRMFARRRILLKKNRHQRAGHGAKNKLKPITILTEKSERFRKKLIERWACEIADFFVKNRVGTVQMENLESMKRKEDSYFNIRLRGFWPYAEMQNKIEFKLKQYGIKVRKVAPNNTSKTCSKCGHLNNYFSFEYRKKNKFPHFKCEKCNFKENADYNAALNISNPKLKSTKEEP

SEQ ID NO: 999 - protein, 725 aa, synthetic construct
SEVEFSHEYWMRHALTLAKRARDEREVPVGAILVLNNRVIGEGWNRAIGLHDPTAHAEIMALRQGGLVMQNYRLIDATLYVTFEPCVMCAGAMIHSRIGRVVFGVRNNKHGAAGSLVNVLDYPGMNHRVEITEGILADECAALLCDFYRMPRQVFNARKKAQSSISLGGSSGGSSGSETPGTSESATPESSGGSSGGSAKNTITKTLKLRIVRPYNSAEVEKIVADEKNSREKIALEKNKDKVKEACSKHLKVAAYCTTQVERNACLFCKARKLDDKFYQKLRGQFPDAVFWQEIGEVFRQLQKQAAEIYNQSLIELYYEIFIKGKGFANASSVEHYLSDVCYTRAAELFKNAAIASGLRNKIKSNFRLKELRNMKSGLPTTKSDNFPIPLVKQKGGQYTGFEISNHNGDFIIKIPFGRWQVKKEINKHRPWEKFDFEQVRKSPKPISLLLSTQRRKRNKGWSKDEGTEAEIRKVMNGDYQTSYIEVKRGSKIGEKSAWMLNLSIDVPKIDKGVDPGIIGGIDVGVKSPLVCAINNASSRYSISDNDLFHFNKKMFARRRILLKKNRHKRAGHGAKNKLKPITIMTEKSKRFRKKLIERWACEIADFFIKNKVGTVQMENLESMKRKEDSYFNIRLRGFWPYAEMQNKIEFKLKQYGIEIRKVAPNNTSKTCSKCGHLNNYFNFEYRKKNKFPHFKCEKCNFKENADYNAALNISNPKLKSTEEP

SEQ ID NO: 1000 - protein, 726 aa, synthetic construct
SEVEFSHEYWMRHALSLAKRARDEREVPVGAVLVLNNRIIGEGWNRAIGLHDPTAHAEIMALRQGGLVMQNYRLTGATLYVTFEPCVMCAGAMVHSRIGRVVFGVRNSKRGAAGSLMNVLNYPGMNHCVEITEGILVDECAALLCDFYRMPRQVLNAQKKAQSSIRSGGSSGGSSGSETPGASGSVTPKSSGGSSAGSTKDTVTKTLKLRIVRPYNSAEVEKIVADEKNNREKIALEKNKDKVKEACSEHLKVAAYCTTQVERSACLFCKARKLDDKFYQKLRSQFPDAVFWQELGEIFRQLQKQTAEIYNQSLIELYYEILIKGKGFANASSVEHYLSDVCYTRAAELFKNAAIASGLRGKVKSNFRLKELKNMRSGLPTTKSDNFPIPLVKQKGGQYTGFEISSHNDDFIIKIPFGRWQVKKEIDKYRPWERFDFEQVRKSPKPISLLLSTQRRKRNKGWSKDEGTEAEIRKVMNGDYQTSYIEVKRGSKIGEKSAWMLNLSIGVPKIDKGVDPSIIGGIDVGVKSPLVCAINNAFSRYSISDNDLFHFNKKMFARRRILLKKSKHKRAGHGAKNKLKPITIMTEKSKRFRKKLIERWACEIADFFIKNKVGTVQMENLESMKRREDSYFNIRLRGFWPYAEMQNKIEFKLKQYGIEIRKVAPNNTSKTCSKCGHLNNYFNFEYRKKNKFPHFKCEKCNFKENADYNAALNISNPKLKSTKEEP

SEQ ID NO: 1001 - protein, 726 aa, synthetic construct
SEVELSHEYWMRHALSLAKRARDEREVPVGAVLVLNNRVIGEGWNRAIGLHDPTAHAEIMALRQGGLVMQNHRLIDATLYVTFEPCVMCAGAMIHSRIGRVVFGVRNSKRGAAGSLMNVLNYPGMNHRVEITEGILTDECAALLCDFYRMPHQVLNAQKKAQSSINSGGSSGGSSGSETPGTSESPTPESSGGSPGGFAKNTITKTLKLRIVRPYNSAEVEKIVADEKNNREKIALEKNKDKVREACSKHLKVAAYCTTQVERSACLFCKARRLDDKFYQKLKGQFPDAVFWQELGEIFRQLQKQAAEIYNQSLIELYYEIFIKGKGFANASSVEHYLSDVCYTRAAELFKNAAIASGLRGKVKSNFRLKELKNMKSGLPTTKSDNFPIPLVKQKGGQYTGFEISSHNDDFIIKIPFGRWRVKKEIDKYRPWEKFDFEQVRKSPKPISLLLSTQRRKRSKGWSKDEGTEAEIRKVMNGDYQTSYIEVKRGSKTGEKSTWMLNLSIDVPKIDKGVDPSIIGGIDVGVKSPLVCAINNAFSRYSISDNDLFRFNKKMFARRRILLKKNRHKRAGHGAKNKLKPITIMTEKSKRFRKKLIERWACEIADFFIKNKVGTVQMENLESMKRKEDSYFNIRLRGFWPYAEMQNKIEFKLKQYGIVVRKVAPNNTSKTCSKCGHLNNYFNFEYRKRNKFPHFKCEKCNFKENADYNAALNISNPKLKGTKEEP

SEQ ID NO: 1002 - protein, 726 aa, synthetic construct
SEVEFSHEYWMRHALTLAKRARDEREVPVGAILVLNNRVIGEGWNRAIGLHDPTAHAEIMALRQGGLVMQNYRLIDATLYVTFEPCVMCAGAMIHSRIGRVVFGVRNNKHGAAGSLVNVLNYPGMNHRVEITEGILADECAALLCDFYRMPRQVFSARKKAQSSINPGGSSGGSSGGKAPGTSESATLESSGGSSGSSAKNTITKTLKLRIVRPYNSAEVEKIVADEKNNREKTALEKNKGKVKEACSKHLKVATYCTTQVERNACLFCKARKLDDEFYQKLRGQFPDAVFWQEIGEIFRQLQKQAAEIYNQSLIELYYEIFIKGKGITNASRVEHYLSDVCYTRAAEQFKNAAIASGLRGKVKSNFRLKELKNMKSGLPTTKSDNFPIPLVKQKGGQYTGFEISSHNDDFIIKIPFGRWQVKKEINKFRPWEKFDFEQVRKSPKPISLLLSTQRRKRNKGWSKDEGTEAEIRKVMNGDYQTSYIEVKRGSKIGEKSAWMLNLSIDVPKIDKGVNPSIIGGIDVGVKSPLVCAINNSSSRYSICDNDLFRFNKKMFARRRILLKKNRHKRAGHGAKNKLKPITILTERSERFRKKLIERWACEIADFFIKNKVGTVQMENLESMKRKEDSYFNIRLRGFWPYAEMQNKIEFKLKQYGIKVRKVAPNNTSKTCSKCGHLNNYFSFEYRKKNKFPHFKCEKCNFKENADYNAALNISNPKLKSTKGEP

SEQ ID NO: 1003 - protein, 725 aa, synthetic construct
SEVGFSHEYWMRHALTLAKRARDEREVPVGAVLVLNNRVIGEGWNRAIGLHDPTAHAEIMALRQGGLVMQNYRLTDATLYVTFEPCVMCAGAMIHSRIGRVVFGVRNSKRGAAGSLMNVLNYPGMNHCVEITEGILVDECAALLCDFYRMPRQVLNAQKKAQSSISPGGSSGGSSGSETPGASGSVTPKSSGGSSGGSAKNTITKTLKLRIVRPYNSAEVEKVVADEKNNREKIALEKNEDKVKEACSKHLKVAAYCTTQVERNACLFCKARRLDDKFYQKLRGQFPDAVFWQEIGEIFRQLQKQAAEVYNQSLVELYYEILIKGKGIANASSVEHYLSDVCYTRAAELFKNAAIASGLRNKIKSNFRLKELRNMKSGLPTTKSDNFPIPLVRQKGGQYTGFEISNHDGDFIIKIPFGRWQEKKEINKHRPWEKFDFEQVRKSPKPISLLLSTQRRKRNKGWSKDEGTEAEIRKVMNGDYQTSYIEVKRGSKIGEKSAWMLNLSIDVPKIDKGVDPSIIGGIDVGVKSPLVCAINNALSRYSISDNDLFHFNKKMFARRRILLRKNRHKRAGHGAKNKLKPITIMTEKSKRFRKKLIERWACEIADFFIKNRVGTVQMENLESMKRKEDSYFNIRLRGFWPYAEMQNKIEFKLKQYGIVVRKVAPNNTSKTCSKCGHLNNYFNFEYRKKNKFPHFKCEKCNFKEDADYNAALNISNPKLSTKGEP

SEQ ID NO: 1004 - protein, 726 aa, synthetic construct
SEVEFSHEYWMRRALTLAKRARDEREVPVGAVLVLNNRVIGVGWNRAVGLHDPTAHAEIMALRQGGLVMQNYRLIEATLYVTFEPCIMCAGAMIHSRIGRVVFGVRNSKRGAAGSLMNVLNYPGMSHRVEITEGILADECAALLCDYYRMPRQVFNARKKVQSSINSGGSSDGGSSSETPGTSESATPESSGGSSGGSAKNTITKTLKLRIVRPYNSAEVEKIVADEKNNREKIALEKNKDKVKEACSEHLKVAAYCTTQVERSACLFCKARKLDDKFYQKLRSQFPDAVFWQEIGEIFRQLQKQAAEIYNQSLIELYYEIFIKGKGFANASSVEHYLSDVCYTRAAELFKNAAIASGLRNKIKSNFRLKELRNMKSGLPTTKSDNFPIPLVKQKGGQYTGFEINSHNDDFIIKIPFGRWQVKKEIDKYRPWEKFDFEQVRKSPKPISLLLSTQRRKRNKGWSKDEGTEAEIRKVMNGDYQTSYIEVKRGSKTGEKSAWMLNLSIDVPKIDKGVDPSIIGGIDVGVKSPLVCAINNAFSRYSISDNDLFRFNKKMFARRRILLKKNRHKRAGHGAKNKLKPISVLTEKSRRFRKKLIERWACEIADFFIKNKVGTVQMENLGSMKSKEDSYFNIRLRGFWPYAEMQNKIEFKLKQYGIEIRKVAPDNTSKTCSKCGHLNNYFNFEYRKKNKFPHFKCEKCNFKEDADYNAALNISNPKLKSTKEEP

SEQ ID NO: 1005 - protein, 726 aa, synthetic construct
SEVEFSHEHWMRHALTLAKRARDEREVPVGAVLVLNNRVIGEGWNRAIGLHDPTAHAEIMALRQGGLVMQNYRLIDATLYVTFEPCVMCAGAMVHSRIGRVVFGVRNSKRGAAGSLMNVLDYPGMNHRVEITEGILADECAALLCDFYRMPRQVFNAQKKARPNINSGGSSGGRSGSEAPGTSESATPESSGGSFGGSAKNTITKTLQLRIVRPYNSAEVEKIVADEKNNREKIALEKNKDKVKEACSKHLKVAAYCTTQVERNACLFCKARKLDDKFYQKLRGQFPDAVFWQELGEILRQLQKQAAEIYNQSLIELYYEIFIKGRGFANASSVEHYLSDVCYTRAAELFKNAAIASGLRGKVKSNFRLKELKNMKSGLPTTKSDNFPIPLVKQKGGQYAGFEISSHNDDFIIKIPFGRWQVKKEIDKYRPWEKFDFEQVRKSPKPISLLLSTQRRKRNKGWSKDEGTEAEIRKVMNGDYQTSYIEVKRGSKIGEKSAWMLNLSIDVPKIDKGVDPSIIGGIDVGVKSPLVCAINNALSRYSISDNDLFHFNKKMFARRRILLRKNRHKRAGHGAKNKLKPITIMTEKSKRFRKKLIERWACEIADFFIKNKVGTVQMENLESMKRKEDSYFNIRLRGFWPYAEMQNKIEFKLKQYGIEIRKVAPNNTSKTCSRCGHLNDYFNFEYRRKNKFPHFKCEKCNFKENADYNAALNISNPKLKSTKEEP

SEQ ID NO: 1006 - protein, 726 aa, synthetic construct
SEVEFSHEYWMRHALTLAKRARDEREVPVGAILVLNNRVIGEGWNRAIGLHDPTAHAEMMALRQGGLVMQNYRLIDATLYVTFEPCVMCAGAMVHSRIGRVVFGVRNSKRGAAGSLMNVLDYPDMGHRVEITEGILADECAALLCDFYCMPRQVFNARKKAQSSINSGGSSDGGSGSETPGTSESATPESTGGSSGGSAKNTITKALKLRIVRPYNSAEVEKIVADEKNNREKIALEKNKDKVKEACSKHLKVAAYCTTQVERNACLFCKARRLDDKFYQKLRGQFPDAVFWQEIGEIFRQLQKQAAEIYNQSLVELYYEIFIKGKGIANASSVEHYLSDVCYTRAAELFKNAAIASGLRNKIKSNFRLKELRNMKSGLPTTKSDNFPIPLVRQKGGQYTGFEISNHNGDFIIKIPFGRWQVKKEISKHRPWEKFDFEQVRKSPKPISLLLSTQRRKRNKGWGKDEGTEAEIRKVMNGDYQTSYIEVKRGSKIGEKSAWMLNLSIDVPKIDKGVDPSIIGGIDVGVKSPLVCAINNALSRYSIGDNDLFHFNKKMFARRRILLRKNRHKRAGHGARNKLKPITVLTEKSERFRKKLIERWACEIANFFIKNKVGTVQMENLESMKRRGDSYFNIRLRGFWPYAEMQSKIEFKLKQYGIKIRKVAPNNTSKTCSKCGHLNNYFNFEFRKKNKFPHFKCEKCNFKEDADYNAALNISNPKLKSTKEEP

SEQ ID NO: 1007 - protein, 726 aa, synthetic construct
SEVEFSHEYWMRHALALAKRARDEREVPVGAVLVLNNRVIGEGWNRAIGLHDPTAHAEIMALRQGGLVTQNYRLIDATLYATFEPCVMCAGAMIHSRIGRVVFGVRNSKRGAAGSLMNVLNYPGMDHRVEITEGILADECAALLCDFYRMPRQVFNARRKAQSSISSGGSSGGSSGSETPGTSKSATLEGSGGSSGGSTKNTVTKTLKLRIVRPYNSAEVEEIVANEKNNREKIALEKNKDKVKEACSRHLKVAAYCTTQVERSACLFCKARKLDDKFYQKLKGQFPDAVFWQEISEIFRQLQKQAAEIYNQSLIELYYEIFIKGKGITNASSVEHYLSDVCYTRAAELFKNAAIASGLRGKIKSNFRLKELKNMKSGLPTTKSDNFPIPLVKQKGGQYTGFEISNHNSDFIIKIPFGRWQVKKEISKYRPWERFDFEQVRKSPKPISLLLSTQRRKRNKGWSKDEGTEAEIRKVMNGDYQTSYIEVKRGSKTGEKGAWMLNLSIDVPKIDKGVDPSIIGGIDVGVKSPLVCAIYNALSRYSISDNDLFRFNKKMFARRRILLKKNRHKRAGHGAKNKLKPISILTGKSERFRKKLIERWACEIADFFIKNKVGTVQMENLESMKRKEDSYFNIRLRGFWPYAEMQNKIEFKLKQYGIEIRKVAPNNTSKTCSKCGHLNNYFNFEYRKKNKFPHFKCEKCNFKENADYNAALNISNPKLKSTKEEP

SEQ ID NO: 1008 - protein, 726 aa, synthetic construct
SEVEFSHEYWMRHALTLAKRARDGREVPVGAVLVLNNRVIGEGWNRAIGLHDPTAHAEIMALRQGGLVTQNYRLIDATLYVTFEPCAMCAGAMVHSRIGRVVFGVRNSKRGAAGSLMNVLNYPGMDHRVEITGGILADECAALLCDFYRMPRRVLNAQKKAQSSINSGGSSGGSSGSVTPGTSESATPESSGGSFGGSAKNIITKTLQLRIVRPYNSAEVEKIVADEKNSREKIALEKNKDKVKEACGKHLKVASYCTTQVERNACLFCKARKLDDKFYQKLRGQFPDAVFWQELGEIFRQLQKQAAEIYNQSLIELYYEIFIKGKGLANASSVEHYLSDVCYTRAAELFKNAAIASGLRGKVKSNFKLKELKSMKSGLPSTKSDNFPIPLVKQKGGRYTGFEISSHNDDLVIKIPFGRWQVKKEIDKYRPWEKFDFEQVRKSPKPISLLLSTQRRKRNKGWSKDEGTEAEIRKVMNGDYQTSYIEVKRGSKIGEKSAWMLNLSIDVPKIDKGVDPSITGGIDVGVKSPLVCAINNASSRYSISDNDLFHFNKKMFARRRILLKKNRHKRAGHGAKNKLKPLTILTGKCKRFRKKLIERWACEIADFFTKNKVGTVQMENLESMKRKEDSYFNTRLRGFWPYAEMQSKIEFKLKQYGIEIRKVAPNNTSKTCSKCGHLNNYFNFEYRKRNKFPRFKCEKCNFKENADYNAALNISNPKLKSPKEEP

SEQ ID NO: 1009 - protein, 726 aa, synthetic construct; identical to SEQ ID NO: 869

SEQ ID NO: 1010 - protein, 726 aa, synthetic construct
SEVEFSHEYWMRHALTLAKRARDEREVPVGAILVLNNRVIGEGWNRAIGLHDPTAHAEIMALRQGGLVMQNYRLTDATLYVTFEPCVMCAGAMVHSRIGRVVFGVRNSKRGAAGSLMNVLNYPGVNHCVEITEGILVDECAALLCDFYRMPRQVLNAQKKAQSSISSGGSSGGCSGSEMPGASESVTPKSSGGSSAGSTKNTITKTLKLRIVRPYNSAEVEKIVADEKNSREKIALEKNKGKVKEACGKHLKVASYCTTQVERNACPFCRARKLDDKFYQKLRGQFPDAVFWQEIGEIFRQLQKQAAEIYNQSLIELYYEIFIKGKGFANASSVEHYLSDVCYTRAAELFKNAAIASGLRGKVKSNFRLKELKNMRSGLPTTKSDNFPIPLVKQKGGQYTGFEISSHNDDFIIKIPFGRWQVKKEIDKYRPWEKFDFEQVRKSPKPISLLLSTRRRKRNKGWSKDEGTEAEIRKVMNGDYQTSYIEVKRGSKTGEKSAWMLNLSIDVPKIDKGVDPSIIGGIDVGVKSPLVCAINNALSRYSISDNDLFHFNKKMFARRRILLKKNRHRRAGHGARNKLKPITVLTEKSKRFRKKLIERWACEIANFFIKNKVGTVQMENLESMKRKEDSYFNIRLRGLWPYAEMQNKIEFKLKQYGIEIRKVAPNNTSKTCSKCGHLNNYFSFEYRKKNKFPHFKCEKCNFKENADYNAALNISNPKLKSTKEEP

SEQ ID NO: 1011 - protein, 726 aa, synthetic construct; identical to SEQ ID NO: 592

SEQ ID NO: 1012 - protein, 726 aa, synthetic construct
SEVEFSHEYWMRHALTLAKRARDEREVPVGAVLVLNNRAIGEGWNRAIGLHDPTAHAEIMALRQGGLVMQNYRLTDATLYVTFEPCVMCAGAMIHSRIGRVVFGVRNSKRGAAGSLMNVLNYPGMNHCVEITEGILVDECAALLCDFYRMPRQVLNAQKKAQSSISSGGSSGGSSGSETPGASGSVTPKSSGGSSAGSTKDTITKTLKLRIVRPYNSAEVEKVVADEKNNREKIAMEKNKDKVKEACSKHLKVASYCTTQVERNACLFCKARKLDDKFYQKLRGQFPDAVFWQELGGIFRQLQKQAAEIYNQSLIELYYEIFIKGKGITNASRVEHYLSDVCYTRAAELFKNAAIASGLRSKVRSNFRLKELKNMKSGLPTTKSDNFPIPLVKQKGGQYTGFEISSHNDDFIIKIPFGRWQVKKEIDKYRPWEKFDFEQVRKSPKPISLLLSTRRRKRNKGWSKDEGTEAEIRKVMNGDYQTSYIEVKRGSKIGEKSAWMLNLSIDVPKIDKGVDPSIIGGIDVGVKSPLVCAINNAFSRYSISDNELFHFNKKMFARRRILLKKNRHKRAGHGAKNKLKPISILTEKSKRFRKKLIERWACEIADFFIKNKVGTVQMENLESMKRKEDSYFNIRLRGFWPYAEMQNKIEFKLKQYGIEIRKVAPNNTSKTCSKCGHLNNYFNFEYRKKNKFPHFKCEKCNFKENADYNAALNISNPMLKSTKEEP

SEQ ID NO: 1013 - protein, 726 aa, synthetic construct
SEVEFSHEYWMRHALTLAKRARDEREVPVGAILVLNNRVIGEGWNRTIGLHDPTAHAEIMALRQGGLVMQNYRLIDATLYVTFEPCVMCAGAMIHSRIGRVVFGVRNSKHGAAGSLVNVLNYPGMNHRVEITEGILADECAALLCDFYRMPRQVFNARKKAQSGINPSGSSGGSSGSVTPGTSESATPESSGGGFGGSAKNTITKTLQLRIVRPYNSAEVEKIVADEKNNREKIALEKNKDKVKEACSKHLKVASYCTTQVERNACLFCKARKLDDKFYQKLRGQFPDAVFWQEIGEIFRQLQKQAAEIYNQSLIELYYEIFIKGRGFANASSVEHYLSDVCYTRAAELFKNAAIASGLRGKVRSNFRLKELKNMKSGLPTTKSDNFPIPLVKQKGGQYTGFEISSHNDDFIIKIPFGRWQVKKEIDKYRPWEKFDFEQVRKSPKPISLLLSTQRRKRNKGWSKDEGTEAEIRKVMNGDYQTSYIEVKRGSKTGEKSAWMLNLSIDVPKIDKGVDPSIIGGIDVGVKSPLVCAINNAFSRYSISDNDLFRFNKKMFARRRILLKKNRHKRAGHGAKNKLKPISILTGKSERFRKKLIERWACEIADFFIKNKVGTVQMENLESMKRKEDSYFNIRLRGFWPYAEMQNKIEFKLKQYGIEIRKVAPNNTSKTCSKCGHLNNYFNFEYRKKNKFPHFKCEKCNFKENADYNAALNISNPKLKSTKEKP

SEQ ID NO: 1014 - protein, 726 aa, synthetic construct
SEVEFSHEYWMRHALTLAKRARDEREVPVGAILVLNNRVIGEGWNRAIGLHDPTAHAEIMALRQGGLVMQNYRLIDATLYVTFEPCVMCAGAMIHSRIGRVVFGVRNSKHGAAGSLVNVLNYPGMNHRVEITEGILADECAALLCDFYRMPRQVFSARRKAQSSISPGGSSGGSSGGETPGSSKSLTPESPGGSSGGSAKNTITKTLKLRIVRPYNSAEVEKIVADEKNNREKIALEKNKDKVKEACGKHLKVAAYCTTQVERNACLFCKARKLDDKFYQKLRGQFPDAVFWQEIGEIFRQLQKQAAEIYNRSLIELYYEIFIKGKGFANASSVEHYLSDVCYTRAAELFKNAAIASGLRGKVKSNFRLKELKSMKSGLPTTKSDNFPIPLVKQKGGQYTGFEISSHNDDFIIKIPFGRWQVKKEIDKYRPWEKFDFEQVRKNPKPISLLLSTQRRKRNKGWSKDEGTEAEIRKVMNGDYQTSYIEVKRGSKIGEKSAWMLNLSIDVPKIDKGVDPSIIGGIDVGVKSPLVCAINNAFSRYSISDNDLFRFNKKVFARRRILLKKNRHKRAGHGTKNKLKPITILTEKSGRFRKKLIERWACEIADFFIKNKVGTVQMENLESMKRKEDSYFNIRLRGFWPYAEMQSKIEFKLKQYGIEIRKVAPNNTSKTCSKCGHLNNYFSFEYRKKNKFPHFKCEKCNFKENADYNAALNISNPKLKSTKEES

SEQ ID NO: 1015 - protein, 726 aa, synthetic construct
SEVEFSHEYWMRHALTLAKRARDEREVPVGAVLVLNNRVIGEGWNRTTGLHDPTAHAEIMALRQGGLVMRNYRLTDATLYVTFEPCVMCAGAMIHSRIGRVVFGVRNSKRGAAGSLMNVLNYPGMNHCVEITEGILVDECAALLCDFYRMPRQVLNAQKKAQSSISPGGSSGGSSGSETPGASESVIPKSSGGSSGGSAKNTITKTLKLRIVRPYNSAEVEKIVADEKNNREKIALEKNKGKVKEACSKHLEVAAYCTTQVERNACLFCKARKLDDKFYQKLRGQFPDAVFWQELGEIFRQLQKQAAEIYNQSLIELYYEIFIKGKGFANASSVEHYLSDVCYTRAAELFKNAAIASGLRGKVKSNFRLKELKNMKSGLPTTKSDNFPIPLVKQKGGQYTGFEISSHNDDFIIKIPFGRWQVRKEIDKYRPWEKFNFEQVRKSPKPISLLLSTQRRKRNKGWSKDEGTEAEIRKVMNGDYQTSYIEVKRGSKIGEKSAWMLNLSIDVPKIDKGVDPSIVGGIDVGVKSPLVCAIDNALSRYSISDNDLFRFNKKMFARRRILLKKNRHRRAGHGAKNKLKPISILTEKSKRFRKKLIERWACEIANFFIKNKVGTVQMENLESMKGREDSYFNIRLRGFWPYAEMQSKIEFKLKQYGIEIRKVAPNNTSKTCSKCGHLNNYFNFEYRKRNKFPHFKCEKCNFKENADYNAALNISNPKLKGTKEEP

SEQ ID NO: 1016 - protein, 726 aa, synthetic construct
SEVEFSHEYWMRHALTLAKRARDEREVPVGAILVLNNRVIGVGWNRAIGLHDPTAHAEIMALRQGGLVMQNYRLIDATLYVTFEPCVMCAGAMIHSRIGRVVFGVRNSKHGAAGSLVNVLNYPGMNHRIEITEGILADECAALLCDFYRMPRQVFNRRKKAQSSINSGCSSGGSSGSETPGTSESATPESSGGGSSGSAKNTITKTLQLRIVRPYNSAEVEKIVADEKNNREKIALEKNKGKVKEACSKHLRVASYCTTQVERNACPFCKARKLDDKFYQKLRGQFPDAVLWQELGEILRQLQKQAAEIYNQSLIELYYEIFIKGRGFANASSVEHYLSDVCYTRAAELFKNAAIASGLRGKVKSNFRLKELKNMKSGLPTTKSDNFPIPLVKQKGGQYTGFEISSHNDDFIIKIPFGRWQVKKEIDKYRPWEKFDFEQVRKSPKPISLLLSTQRRKRNKGWSKDEGTEAEIRKVMNGDYQTSYIEVKRGSKIGEKSAWMLNLSIDVPKIDKGVDPSIIGGIDVGVKSPLVCAINNAFSRYSISDNDLFHFNKKMFARRRILLKKNRHKRAGHGAKNKLKPISILTEKSKRFRKKLIERWACEIADFFIKNKVGIVQMENLESMKRKEDSYFNIRLRGFWPYAEMQNKIEFKLKQYGIEIRKVAPNNTSKTCSKCGHLNNYFNFEYRKKNKFPHFKCEKCNFKENADYNAALNISNPMLKSTKEEP

SEQ ID NO: 1017 - protein, 726 aa, synthetic construct
SEVEFSHEYWMRHALTLAKRARDEREVPVGAVLVLNNRVIGEGWNRVIGLHDPTAHAEIMALRQGGLVMQNYRLIDATLYVTFEPCVMCAGAMIHSRIGRVVFGVRNNKHGAAGSLVNVLNYPGMNHRVEITEGILADECAALLCDFYRMPRQVFNARKKAQSSINPGGSSGGSNGSETPGTSESATPESSGGSSGSSAKNTITKTLKLRIVRPYNSAEVEKIVADEKNNREKIALEKNKDKVKEACSKHLKVASYCTTQVERNACPFCKARKLDDKFYQKLRGQFPNAVFWQELGEILRQLQKQAAEIYNQSLIELYYEIFIKGRGFANAGSVEHYLSDVCYTRAAELFKNAAIASGLRGKVKGNFRLKELKNMKSGLPTTKSDNFPIPLVKQKGGQYTGFEISSHDDDFIIKIPFGRWQVKKEIDKYRPWEKFDFEQVRKSPKPISLLLSTQRRKRNKGWSKDEGTEAEIRKVLNGDYQTSYIEVKRGSKTGEKSAWMLNLSINVPKIDKGVDPSIIGGIDVGVKSPLVCAINNAFSRYSISDNDLFRFNKKMFARRRILLKKNRHKRAGHGAKNKLKPISILTGKSERFRKKLIERWACEIADFFIKNKVGTVQMENLESMKRKEDSYFNIRLRGFWPYAEMQNKIEFKLKQYGIEIRKVAPNNTSKTCSKCGHLNNYFNFEYRKKNKFPHFKCEKCNFKENADYNAALNISNPKLKSTKEKP

SEQ ID NO: 1018 - protein, 726 aa, synthetic construct
SEDEFSHEYWMRHALTLAKRARDGREVPVGAVLVLNNRVIGEGWNRAIGLHDPTAHAEIMALRQGGLVMQNYRLIDATLYVTFEPCVMCAGAMVHSRIGRVVFGVRNSKRGAAGSLMNVLDHPGMGHRVEITEGILADECAALLCDFYCMPRQVFNAQKRAQSSINSGGSSGGSSGSETPGTSESATPESSGGGSSGSAKNTITKTLQLRIVRPYNSAEVEKIVADEKNNREKIALEKNKDKVKEACSKHLKVASYCTTQVERNACPFCKARKLDDKFYQKLRGQFPDAVFWQELGEILRQLQKQAAEIYNQSLIELYYEIFIKGKGFANASSVEHYLSDVCYTRAAELFKNAAIASGLRGKVKSNFRLKELKSMKSGLPTTKSDNFPIPLVKQKGGQYTGFEISSHNDDFIVKIPFGRWQVKKEIDKYRPWEKFDFEQVRKSPKPISLLLSTQRRKRNKGWSKDEGTEAEIRRVMNGDYQTSYIEVKRGSKIGEKSAWMLNLSIDVPKIDKGVDPSIIGGIDVGVRSPLVCAINNAFSRYSISDNDLFRFNKKMFARRRILLKKNRHKRAGHGAKNKLRPITILTEKSRRFRKKLIERWACEIADFFIKNKVGTVQMENLGSMKRKEDSYFNIRLRGFWPYAEMQNKIEFKLKQYGIEIRKVAPDNTSKTCSKCGHLNNYFNFEYRKKNKFPHFKCEKCNFKEDADYNAALNISNPKLKSTKEES

SEQ ID NO: 1019 - protein, 726 aa, synthetic construct
SEVEFSHEYWMRHALTLAKRARDEREVPVGAILVLNNRVIGEGWNRAIGLHDPTAHAEIMALRQGGLVMQNYRLTDATLYVTFEPCVMCAGAMIHSRIGRVVFGVRNSKRGAAGSLMNVLNYPGMNHCVEITEGILVDECAELLCDFYRMPRQVLNARKKAQSSINSGGSSGGSSGSETPGTSESATPKSSGGSSGGSAKNTITKALKLRIVRPYNSAEVEKIVADEKNNRERIALEKNKDKVKEACSKHLKVAAYCTTQVERNACLFCKARKLDDKFYQKLRGQFPDAVFWQELGEIFRQLQKQAAEIYNQSLIELYYEIFIKGRGFANASSVEHYLSDVCYTRAAGLFKNAAIASGLRGKVKSNFRLKELKNMKSGLPTTKSDNFPIPLVKQKGGQYAGFEISSHNDDFIIKIPFGRWQVKKEVDKYRPWEKFDFEQVRKSPKPISLLLSTQRRKRNKGWSKDEGTEAEIRKVMSGDYQTSYIEVKRGSKIGEKSAWMLNLSIDVPKIDKGVDPSIIGGIDVGVKSPLVCAINNAFSRYSISDNDLFHFNKKMFARRRILLKKNRHKRAGHGAKNKLKPLTILTGKSKRFRKKLIERWACEIADFFIKNKVGTVQMENLESMKRKEDSYFNIRLRGFWPYAEMQNKIEFKLKQYGIEIRKVAPNNTSKTCSKCGHLNNYFNFEYRKRNKFPRFKCEKCNFKENADYNAALNISNPKLKSPKEEP

SEQ ID NO: 1020 - protein, 726 aa, synthetic construct
SEVEFSHEYWMRHALTLAKRARDEREVPVGAILVLNNRVIGEGWNCAIGLHDPTAHAEIMALRQGGLVMQNYRLIDATLYVTFEPCIMCAGAMIHSRIGRVVFGVRNSKRGAAGSLMNVLNYPGMNHRVEITEGILADECAALLCDYYRMPRQVFNARKKAQSSINSGGSSDGGSGSETPGTSESATPESSGGSSSGSAKNTITKTLQLRIVRPYNSAEVEKIVADEKNNREKIALEKNKDKVKEACSKHLKVASYCTTQVERNACPFCKARKLDDKFYQKLRGQFPDAVFWQELGEILRQLQKQAAEIYNQSLIELYYEIFIKGRGFANASSVEHYLSDVCYTRAAELFKNAAIASGLRGKVKGNFRLKELKNMKSGLPTTKSDNFPIPLVKQKGGQYTGFEISSHNDDFIIKIPFGRWQVKKEIDKYRPWEKFDFEQVRKSPKPISLLLSTQRRKRNKGWSKDEGTEAEIRKVMNGDYQTSYIEVKRGSKIGEKSAWMLSLSIDVPKIDKGVDPSTIGGIDVGVKSPLVCAINNAFSRYSISDNDLFRFNKKMFARRRILLKKNRHKRAGHGAKNKLKPISILTEKSKRFRKKLIERWACEIADFFIKNKVGTVQMENLESMKRKEDSYFNIRLRGFWPYAEMQGKIEFKLKQYGIKVRKVAPNNTSKTCSKCGHLNNYFSFEHRKKNKFPHFKCEKCDFKEDADYNAALNISNPKLKSTKEEP

SEQ ID NO: 1021 - protein, 726 aa, synthetic construct
SEVEFSHEYWMRHALTLAKRARDEREVPVGAVLVLNNCVIGEGWNRAIGLHDPTAHAEIMALRQGGLVMQNYRLTDATLYVTFEPCVMCAGAMIHSRIGRVVFGVRNSKRGAAGSLMNVLNYPGMNHCVEITEGILMDECAALLCDFYRMPRQVLSAQKKAQSSINSGDSSDGGSGSETPGTSESATPESSGGSSGGSAKNTITKTLKLRIVRPYNSAEVEKIVADEKDNREKIALEKNKDKVKEACSKHLKVAAYCTTQVERNACLFCKARRLDDKFYQKLRGQFPDAVFWQEIGEIFRQLQKQAAEIYNQSLVELYYEILIKGKGIANASSVEHYLSDVCYTRAAELFKNAAIASGLRNKIKSNFRLKELRNMKSGLPTTKSDNFPIPLVKQKGGQYTGFEISSHNDDFIIKIPFGRWRVKKEIDKYRPWEKFDFEQVRKSPKPISLLLSTQRRKRNKGWGKDEGTEAEIRKVMNGDYQTSYIEVKRGSKIGEKSAWMLNLSIDVPKIDKGVDPSIIGGIDVGVKSPLVCAINNALSRYSISDNDLFHFNKKMFARRRILLRKNRHKRAGHGTKNKLKPITILTEKSGRFRKKLIERWACEIANFFIKNKVGTVQMENLESMKRKEDSYFNIRLRGFWPYAEMQNKIEFKLKQYGIKVRKVAPNNTSKTCSKCGHLNNYFSFEYRKKNKFPHFKCEKCNFKENADYNAALNISNPKLKSTKEEP

SEQ ID NO: 1022 - protein, 726 aa, synthetic construct
SEVEFSHEYWMRHALTLAKRARDEREVPVGAVLVLNDRVIGEGWNRAIGLHDPTAHAEIMALRQGGLVMQNYRLADATLYVTFEPCVMCAGAMIHSRIGRVVFGVRNSKHGAAGSLVNVLNYPGMNHRVEITEGILADECAALLCDFYRMPRQVFNARKKAQSSINPSGSSGGSSGSVTPGTSESATPESSGGGFGGSAKNTITKTLQLRIVRPYNSAEVEKIVADEKNNREKIALEKNKDKVKEACSKHLKVASYCTTQVERNACLFCKARKLDDKFYQKLRGQFPDAVFWQELGEIFRQLQKQAAEIYNQSLIELYYEIFIKGKGLANASSVEHYLSDVCYTRAAELFKNAAIASGLRGKVKSNFRLKELKSMKSGLPSTKSDNFPIPLVKQRGGQYTGFEISSHNDDFIIKIPFGRWQAKKEIDKYRPWEKFDFEQVRKSPKPISLLLSTQRRKRNRGWSKDEGTEAEIRKVMNGDYQTSYIEVKRGSKTGEKSAWMLNLSIDVPRIDKGVDPSIIGGIDVGVKSPLVCAINNAFSRYSISDNDLFRFNKKMFARRRILLGKNRHKRAGHGVKNKLKPITILTEKSGRFRKKLIERWACEIADFFVKNKVGTVQMENLESMKRKEDSYFNIRLRGFWPYAEMQNKIEFKLKQYGIKVRKVAPNNTSKTCSKCGHLNNYFSFEYRKKNKFPHFKCEKCNFKENADYNAALNISNPKLKSTKEEL

SEQ ID NO: 1023 - protein, 726 aa, synthetic construct
SEVEFSHEYWMRHALTLAKRARDEREVPVGAILVLNNRVIGVGWNRAVGLHDPTAHAEIMALRQGGLVMQNYRLIEATLYVTFEPCIMCAGAMIHSRIGRVVFGVRNSKRGAAGSLMNVLNYPGMDHRVEITEGILADECAALLCDYYRMPRQVFNARKKAQSSINSGGSSDGGSGSETPGTCESVTPESSGGSSGGSAKNTITKTLKLRIVRPYNSAEVEKIVADEKNNREKIALEKNKDKVKEACSKHLKVAAYCTTQVERNACLFCKARKLDDKFYQKLRGQFPDAVFWQEIGEVFRQLQKQAAEIYNQSLIELYYEIFIKGKGFANASSVEHYLSDVCYTRAAELFKNAAIASGLRGKVKSNFRLKELKNMKSGLPTTKSDNFPIPLVKQKGGQYTGFEISSHNDDFIIKIPFGRWQVKKEINKFRPWEKFDFEQVRKSPKPISLLLSTQRRKRNKGWSKDEGTEAEIRKVMNGDYQTSYIEVKRGSKIGEKSAWMLNLSIDVPKIDKGVDPSIVGGIDVGVKSPLVCAINSALGRYSISDNDLFHFNKKMFARRRILLKKNGHKRAGHGARNKLKPITVLTEKSKRFRKKLIERWACEIANFFIKNRVGTVQMENLESMKRKEDSYFNIRLRGFWPYAEMQNRIEFKLKQYGIEIRKVAPNNTSKTCSKCGHLNNYFNFEYRKKNKFPHFKCEKCCFKEDADYNAALNISNPKLKSTKEEP

SEQ ID NO: 1024 - protein, 726 aa, synthetic construct
SEVEFSHEYWMRRALTLAKRARDEREVPVGAVLVLNNRAIGVGWNRAVGLHDPTAHAEIMALRQGGLVMQNYRLTDATLYVTFEPCVMCAGAMIHSRIGRVVFGVRNSKRGAAGSLMNVLNYPGMNHCVEITEGILVDECAALLCDFYRMPRQVLNAQKKAQSSISSGGSSGGSSCSETPGASESVTPKSSGGSSAGSTKSTITKTLKLRIVRPYNSAEVEKIVADEKNSREKIALEKNKDKVKEACSEHLKVAAYCTTQVERNACLFCKARKLDDRFYQKLRGQFPDAVFWQEIGEIFRQLQKQAAEIYNQSLIELYYEIFIKGKGFANASSVEHYLSDVCYTRAAELFKNAAIASGLRGKVKSNFRLKELKNMKSGLPTTKSDNFPIPLVRQKGGQYTGFEISNHDGDFIIKIPFGRWQVKKEINKHRPWEKFDFEQVRKSPKPISLLLSTQRRKRNKGWSKDEGTEAEIRKVMNGDYQTSYIEVKRGSKIGEKSAWMLNLSIDVPKIDKGVDPSIIGGIDVGVKSPLVCAINNAFSRYSISDNELFHFNKKMFARRRILLKKNRHKRAGHGAKNKLKPISVLTEKSGRFRKKLIERWACEIADFFIKNKVGTVQMENLGSMKRKEDSYFNIRLRGFWPYAEMQNKIEFKLKQYGIEIRKVAPNNTSKTCSRCGHLNNYFSFEYRKKNKFPHFKCEKCNFKEDADYNAALNISNPKLKSTKEEP

SEQ ID NO: 1025 - protein, 726 aa, synthetic construct
SEVEFSHEYWMRHALTLAKRARDVREVPVGAVLVLNNRVIGEGWNRAIGLHDPTAHAEIMALRQGGLVMQNYRLIDATLYVTFEPCVMCAGAMIHSRIGRVVFGVRNNKHGAAGSLVNVLNYPGMNHRVEITEGILADECAALLCDFYRMPRQVFNARKKAQSSINPGGSSGGSSGSETPGTSESPTPGSSGGSSGGSAKNTITKTLKLRIVRPYNSAEVEKIVAEEKNNREKIALEKNKDKVKEACSKHLKVASYCTTQVERNACLFCKARKLDDKFYQKLRGQFPDAVFWQELGEIFRQLQKQAAEIYNQSLIELYYEIFIKGKGFANASSVEHYLSDVCYTRAAELFKNAAIASGLRGKVKSNFRLKELKNMKSGLPTTKSDNFPIPLVKQKGGQYTGFEISSHNDDFIIKIPFGRWQVKKEIDKYRPWEKFDFEQVRKSPKPISLLLSTQRRKRNKGWSKDEGTEAEIRKVMNGDYQTSYIEVKRGSKIGEKSAWMLNLSIDVPKIDKGVDPNIIGGIDVGVKSPLVCAINNAFNRYSISDNNLFHFNKKMFARRRILLKKNRHKRAGHGAKNKLKPISILTEKSERFRKKLIERWACEIADFFIKNKVGTVQMENLESMKRKEDSYFNIRLRGFWPYAEMQNKIEFKLKQYGIVVRKVAPNNTSKTCSECGHLNNYFNFEYRRKNKFPHFKCEKCNFKENADYNAALNISNPKLKSTKEEP

SEQ ID NO: 1026 - protein, 726 aa, synthetic construct
SEVEFSHEYWMRRALTLAKRARDEREVPVGAVLVLNNRVIGVGWNRAVGLHDPTAHAEIMALRQGGLVMQNYRLTDATLYVTFEPCVMCAGAMIHGRIGRVVFGVRNSKRGAAGSLMNVLNYPGMNHCVEITEGILVDECAALLCDFYRMPRRVFNARKKAQSSISSGGSSGGSSGGDTLGASEGVTPKSSVGSSASSTKNTITKTLKLRIVRPYNSAEVEKIVADEKDNREKIALEKNKDKVKEACSKHLKVAAYCTTQVERNACLFCKARKLDDKFYQKLRGQFPDAVFWQEIGEIFRQLQKQAAEIYNQSLIELYYEIFIKGKGFANASSVEHYLSDVCYTRAAGLFKNAAIASGLRGKVKSNFRLKELKNMKSGLPTTKSDNFPIPLVKQKGGQYTGFEISSHNDDFIIKIPFGRWQVKKEIDKYRPWEKFDFEQVRKSPKPISLLLSTRRRKRNKGWSKDEGTEAEIRKVMNGDYQTSYIEVKRGSRIGEKSAWMLSLSIDVPKIDRGVDPSIIGGIDVGVKSPLVCAINNALSRYSISDNDLFHFNKKMFARRRILLKKNRHRRAGHGARNKLKPITVLTEKSKRFRKKLIEKWACEIADFFIKNKVGTVQMENLESMKRREDSYFNIRLRGFWPYAEMQNKIEFKLKQYGIEIRKVAPNNTSKTCSKCGHLNNYFNFEYRKKNKFPHFKCEKCNFKENADYNAALNISNPKLKSTKEEP

SEQ ID NO: 1027 - protein, 726 aa, synthetic construct
SEVEFSHEYWMRHALTLAKRARDEREVPVGAILVLNNRVIGEGWNRAIGLHDPTAHAEIMALRQGGLVMQNYRLVNATLYVTFEPCVMCAGAMIHSRIGRVVFGVRNSRRGAAGSLMNVLDYPGMNHRVEITEGILADECAALLCDFYRMPRQVLNAQKKAQSSFNSGGLSGGSSSSETPGTSGSATPEGSGGSSGGSAKNTITKTLKLRIVRPYNSAEVEKIVADEKNNREKIALEKNKDKVKEACSKHLKVASYCTTQVERNACLFCKARRLDDKFYQKLRGQFPDAVFWQELGEIFRQLQKQAAVIYNQGLIELYYEIFIKGKGIANASRVEHYLSNVCYTRAAELFKNAAIASGLRGKVKSNFRLKELRNMKSGLPTTKSDNFPIPLVRQKGGQYTGFEISNHDGDFIIKIPFGRWRVKKEINKHRPWEKFDFEQVRKSPKPISLLLSTQRRKRNKGWSKDEGTEAEIRKVMNGDYQTSYIEVKRGSKIGEKSAWMLNLSIDVPKIDKGVDPGIIGGIDVGVKSPLVCAINSASSRYSISDNDLFHFNKKMFARRRILLKKNGHKRAGHGAKNKLKPITIMTEKSKRFRKKLIERWACEIADFFIKNKVGTVQMENLEGMRRKEDSYFNIRLRGFWPYAEMQNKIEFKLKQYGIGIRKVAPNNTSKTCSKCGHLNNYFNFEYRKKNKFPHFKCEKCNFKENADYNAALNISNPKLKSTKEEH

SEQ ID NO: 1028 - protein, 726 aa, synthetic construct
SEVEFSHEYWMRHALTLAKRARDEREVPVGAVLVLNNRVIGEGWNRAIGLHDPTAHAEIMALRQGGLVMQNYRLIDATLYVTFEPCVMCAGAMIHSRIGRVVFGVRNSKHGAAGSLVNVLNYPGMNHRVEITEGILADECAALLCDFYRMPRQVFNARKKAQSSINSGGSSGGSSGSETPSTSESATPESSGGSSGGSAKNTITKTLKLRIVRPYNSAEVEKIVADEKNNREKIALEKNKDKVKEACSKHLKVASYCTTQVERNACLFCKARKLDDKFYQKLRGQFPDAVFWQELGEIFRQLQKQAAEVYNQSLIELYYEIFIKGKGFANASSVEHYLSDVCYTRAAELFKNAAIASGLRGKVKSNFRLKELKNMKSGLPTTKSDNFPIPLVKQKGGQYTGFEISSHNDDFIIKIPFGRWQVKKEIDKYRPWEKFDFEQVRKSPKPINLLLSTQRRKRNKGWSKDEGTEAEIRKVMNGDYQTSYIEVKRGSKTGEKSAWMLNLSIDVPKIDKGVDPSIIGGIDVGVKSPLVCAINNALSRYSISDNDLFHFNKKMFARRRILLKKSRHKRAGHGAKNKLKPITILTEKSRRFRKKLIERWACEIADFFIKNKVGTVQMENLESMKRKEDSYFNIRLRGFWPYAEMQNKIEFKLRQYGIEIRKVAPNNTSKTCSKCGHLNNYFNFEYRKKNKFPHFKCEKCNFKENADYNAALNISNPKLKSTKEEP

SEQ ID NO: 1029 - protein, 726 aa, synthetic construct
SEVEFSHEHWMRHALTLAKRARDEREVPVGAVLVLNNRVIGEGWNRAIGLHDPTAHAEIMALRQGGLVMQNYRLTDATLYVTFEPCVMCAGAMIHSRIGRVVFGVRNSKRGAAGSLMNVLNYPGMNHCVEITEGILMDECAALLCDFYRMPRQVLNAQKKAQSSISSGGSSGGSSGSETPGAGESVTPKSSVGSSAGSTKNTITKTLKLRIVRPYNSAEVERIVADEKNNREKTALEKNKDKVKEACSRHLKVAAYCTTQVERNACLFCKARKLDDKFYQKLRGQFPDAVFWQEVGEIFRQLQKQAAEIYNRSLIELYYEIFIKGKGFANASSVEHYLSDVCYTRAAELFRNAAIASGLRGKVKSNFRLKELKNMKSGLPTTKSDNFPIPLVRQKGGQYTGFEISSHNDDFIIKIPFGRWQVKEEIDKYRPWEKFDFEQVRKNPKPISLLLSTLRRKRNKGWSKDEGTEAEIRKVMNGDYQTSYIEVKRGSKIGEKSTWMLNLSIDVPKIDKGVDPSIVGGIDVGVKSPLVCAINNAFSRYSISDNDLFHFNKKMFARRRILLKKNRHKRAGHGAKNKLKPISILTEKSKRFRKKLIERWACEIADFFIKNKVGTVQMENLESMKRKEDNYFNIRLRGFWPYAEMQNKIEFKLKQYGIEIRKVAPNNTSKTCSKCGHLNNYFNFEYRKKNKFPHFKCEKCNFKENADYNAALNISNPELKSTKEEP

SEQ ID NO: 1030 - protein, 726 aa, synthetic construct
SEVEFSHEHWMRHALTLAKRARDEREVPVGAVLVLNNRVIGEGWNRTTGLHDPTAHAEIMALRQGGLVMQNHRLVDATLYVTFEPCVMCAGAMIHGRIGRVVFGVRNSKRGAAGSLTNVLNYPGMNHRVEITEGILVDECAALLCDFYRMPRQVFNAQKKAQSTINSGGSSGGSSGSETPGTSESPTPESSGGSPGGSAKNTITKTLKLRIVRPYNSAEVEKIVADEKNNREKIALEKNKDKVKEACSKHLKVAAYCTTQVERNACLFCKARKLDDKFYQKLRGQFPDAVFWQEIGEIFRQLQKQAAEIYNQSLIELYYEIFIKGKGFANASSVEHYLSDVCYTRAAELFKNAAIASGLRGKVKSNFRLKELKNMKSGLPTTKSDNFPIPLVKQKGGQYTGFEISSHNDDFIIKIPFGRWQVKEEIDKYRPWEKFDFEQVRKSPKPISLLLSTQRRKRNKGWSKDEGTEAEIRKVMNGDYQTSYIEVKRGSKIGEKSAWMLNLSIDVPKIDKGVDPSIIGGIDVGVKSPLVCAINNAFSRYSISDNDLFHFNKKMFARRRILLKKNRHKRAGHGTKNKLKPITILTEKSGRFRKKLIERWACEIANFFIKNKVGTVQMENLESMKRKEDSYFNIRLRGFWPYAEMQNKIEFKLKQYGIKIRKVAPNNTSKACSKCGHLNNYFSFEYRKKNKFPHFKCEKCNFKEDADYNAALNISNPKLKSTKEEP

SEQ ID NO: 1031 - protein, 726 aa, synthetic construct
SEVEFSHEYWMRHALSLAKRARDEREVPVGAVLVLNNRIIGEGWNRAIGLHDPTAHAEIMALRQGGLVMQNYRLTDATLYVTFEPCVMCAGAMIHSRIGRVVFGVRNNKHGAAGSLVNVLNYPGMNHRVEITEGILADECAALLCDFYRMPRQVFNARKKAQSSINSGGSSGGSSGSETLGTSESATPESSGGSSGGSAKNTITKTLQLRIVRPYNSAEVEKIVADEKNNRERIALEKNKDKVREACSKHLKVASYCTTQVERNACLFCKARRLDDKFYQKLRGQFPDAVFWQELGEIFRQLQKQAAEVYNQSLVELYYEILIKGKGIANASSVEHYLSDVCYTRAAELFKNAAIASGLRNKIKSNFRLKELRNMKSGLPTTKSDNFPIPLVRQKGGQYTGFEISSHDGDFIIKIPFGRWQVKKEIDKYRPWEKFDFEQVRKSPKPISLLLSTRRRKRNKGWSKDEGTEAEIRKVMNGDYRTSYIEVKRGSKTGEKSAWMLNLSIDVPKIDKGVDPSIIGGIDVGVKSPLVCAINNAFSRYSISDNDLFRFNKKMFARRRILLGKNRHKRAGHGVKNKLKPITILTEKSGRFRKKLIERWACEIADFFIKNKVGTVQMENLESMKRKEDSYFNIRLRGFWPYAEMQNKIEFKLKQYGIEIRKVAPNNTSKTCSKCGHLNSYFNFEYRKKNKFPHFKCEKCNFKENADYNAALNISNPKLKSTKEEP

SEQ ID NO: 1032 - protein, 726 aa, synthetic construct
SEAESSHEYWMRRALTLAERARDEREVPVGAVLVLNNRVIGVGWNRAIGLHDPTAHAEIMALRQGGLVTQNYRLIDATLYVTFEPCIMCAGAMIHSRIGRVVFGVRNSKRGAAGSLMNVLDYPGMNHRVEITEGILAGECAALLCDFYRMPRQVFNAQKKAQSNINPGGSSGGSSGSETPGTSESPTPESSGGSSGGSAKSTITKTLKLRIVRPYNSAEVEKIVADEKNNREKIALEKNKDKVKEACSKHLKVAAYCTTQVERNACLFCKARKLDDRFYQKLRGQFPDAVFWQEIGEIFRQLQRQAAEIYNQSLIELYYEIFIKGKGFANASSVEHYLSDVCYTRAAELFKNAAIASGLRGKVKSNFRLKELRNMKSGLPTTKSDNFPIPLVKQKGGQYTGFEIRSHNDDFIIKIPFGRWQVKKEIDRYRPWEKFDFEQVRKSPKPISLLLSTQRRKRNKGWSKDEGTEAEIRKVMNGDYQTSYIEVKRGSKIGEKNAWMLNLSIDVPKIDKGVDPSIIGGIDVGVKSPLVCAINNASSRYSISDNDLFHFNKKMFARRRILLKKNGHKRAGHGTKNKLKPITIMTEKSKRFRKKLIERWACEIADFFIKNKVGTVQMENLESMKRKEDSYFNIRLRGFWPYAEMQNKIEFKLKQYGIVVRRVAPNNTSKTCSKCGHLNNYFNFEYRKKNKFPHFKCEKCNFKENADYNAALNISNPKLKSTKEGP

SEQ ID NO: 1033 - protein, 726 aa, synthetic construct
SEVEFSHEYWMRHALTLAKRARDEREVPVGAVLVLNNRVIGEGWNRTTGLHDPTAHAEIMALRQGGLVMQNHRLVDATLYVTFEPCVMCAGAMIHSRIGRVVFGIRNSKRGAAGSLTNVLNYPGMSHRVEITEGILADECAALLCDFYRMPRQVFNAQKKAQSNINPGGSSGGSSGGETPGTSKSATPGSSGGSSGGSAKNTITKTLKLRIVRPYNSAEVEKIVADEKNNREKIALEKNKDKVKEACSEHLKVAAYCTTQVERNACLFCKARKLDDKFYQKLRGQFPDAVFWQEIGEIFRQLQKQAAEIYNQSLIELYYEIFIKGKGFANASSVEHYLSDVCYTRAAELFKNAAIASGLRGKVKSNFRLKELKNMKSGLPTTKSDNFPIPLVKQKGGQYTGFEISSHNDDFIIKIPFGRWQVKKEIDKYRPWEKFDFEQVRKSPKPISLLLSTQRRKRNKGWSKDEGTEAEIRKVMNGDYQISYIEVKRGSKIGEKSAWMLNLSIDVPKIDKGVDPRIIGGIDVGVKSPLVCAINNAFSRYSISDNDLFHFNKKMFARRRILLKKNRHKRAGHGAKNKLKPISILTGKSERFRKKLIERWACEIADFFIKNKVGTVQMENLESMRRKEDSYFNIRLRGFWPYAEMQNKIEFKLKQYGIEIRKVAPNNTSKTCSKCGHLNNYFNFEYRKKNKFPHFKCEKCNFKENADYNAALNISNPKLKSTKGEP

SEQ ID NO: 1034 - protein, 726 aa, synthetic construct
SEVEFSHEYWMRHALTLAKRARDEREVPVGAVLVLNNRVIGEGWNRTTGLHDPTAHAEIMALRQGGLVMRNYRLTDATLYVTFEPCVMCAGAMIHSRIGRVVFGVRNSKRGAAGSLMNVLNYPGMNHCVEITEGILVDECAALLCDFYRMPRQVLNAQRKAQSSISPGGSSGGSSGSVTPGASESVTPKSSGGSSGGSAKDTITKTLKLRIVRPYNSAEVEKIVADEKNNREKIALEKNKGKVKEACSKHLEVAAYCTTQVERNACLFCKARRLDDKFYQRLRGQFPDAVFWQELGEIFRQLQKQAAEIYNQSLIELYYEIFIKGKGFANASSVEHYLSDVCYTRAAELFKNAAIASGLRGKIKSNFRLKELKNMKSGLPTTKSDNFPIPLVKQKGGQYTGFEISNHNGDFIIKIPFGRWQVKKEIDKYRPWEKFDFEQVRKSPKPISLLLSTQRRKRNKGWSRDEGTEAEIKKVMNGDYQISYIEVKRGSKIGEKSAWMLNLSVDVPKIDKGVDPSIIGGIDVGVKSPLVCAINNALSRYSISDNDLFHFNKKMFARRRILLKKNRHRRTGHGARNKLKPITVLTEKSERFRKKLIERWACEIANFFIKNKVGTVQMENLESMKRREDSYFNIRLRGLWPYAEMQNKIEFKLKQYGIEVRKVAPDNTSKTCSKCGHLNNYFNFEYRKKNKFPLFKCEKCNFKENADYNAALNISNPKLKSTKGEP

SEQ ID NO: 1035 - protein, 726 aa, synthetic construct
SEVEFSHEYWMRHALTLAKRARDEREVPVGAILVLNNRVIGEGWNRAIGLHDPTAHAEIMALRQGGLVMRNYRLVDATLYVTFEPCVMCAGAMIHSRIGRVVFGVRNNKHGAAGSLVNVLNYPGMNHRVEITEGILVDECAALLCDFYRMPRQVLNARKKAQSSINPGGSSGGSSGSETPGTSESATPESSGGSSGGSAKNTITKTLKLRIVRPYNSAEVEKIVADEKNNREKIALEKNKDKVKEACSKHLKVAAYCTTQVERNACLFCKARKLDDKFYQKLRGQFPDAVFWQEIGEIFRQLQKQAAEIYNQSLIELYYEIFIKGKGFANASSVEHYLSDVCYTRAAELFKNAAIASGLRGKVKSNFRLKELKNMRSGLPTTKSDNFPIPLVKQKGGQYAGFEISSHNDDFIIKIPFGRWQVKKEIDKYRPWEKFDFEQVRKSPKPISLLLSTRRRKRNKGWSKDEGTEAEIRKVMNGDYQTSYIEVKRGSKIGEKSAWMLNLSIDVPKIDKGVDPSIIGGIDVGVKSPLVCAINNAFGRYSISDNDLFHFNKKMFARRRILLKRNRHKRAGHGTKNKLKPITILTEKSGRFRKKLIERWACEIANFFIKNKVGIVQMENLESMKRKEDSYFNIKLRGFWPYAEMQNKIEFKLKQYGIEIRKVAPNNTSKTCSRCGHLNNYFSFEYRKKNKFPHFKCEKCNFKEDADYNAALNISNPKLKSTKEEP

SEQ ID NO: 1036 - protein, 726 aa, synthetic construct
SEVEFSHEYWMRHALTLAKRARDEREVPVGAVLVLNNRVIGEGWNRTTGLHDPTAHAEIMALRQGGLVMQNHRLVDATLYVTFEPCVMCAGAMIHSRIGRVVFGVRNSKRGAAGSLVNVLNYPGMNHRVEITEGILADECAALLCDFYRMPRQVFNARRKAQPSINPGGSSGGSSGSETPGTSESATPESSGGSSGGSAKNTITKTLKLRIVRPYNSAEVEKIVADEKNNREKIALEKNRDKVKEACSKHLKVAAYCTTQVERNACLFCKARKLDDKFYQKLRGQFPDAVFWQEISEIFRQLQKQAAEIYNQSLIELYYEIFIKGKGFANASSVEHYLSDVCYTRAAELFKNAAIASGLRGKVKSNFRLKELKNMKSGLPTTKSDNFPIPLVKQKGGQYTGFEISSHNSDFIIKIPFGRWQEKEEIDKYRPWEKFDFEQVRKSPKPISLLLSTQRRKKNKGWSKDEGTEAEIRRVMNGDYRTSYIEVKRGSKIGEKSAWMLNLSIDVPKIDKGVDPSIIGGIDVGVKSPLVCAINNAFSRYSISDNDLFRFNKKMFARRRILLRKNRHKRAGHGAKNKLKPISILTGKSERFRKKLIERWACEIADFFIRNKVGTVQMENLESMKRKEDSYFNIRLRGFWPYAEMQNKIEFKLKQYGIEIRKVAPNNTSKTCSKCGHLNNYFNFEYRKKNKFPHFKCEKCNFKENADYNAALNISNPKLKSTKEEP

SEQ ID NO: 1037 - protein, 726 aa, synthetic construct
SEVEFSHEYWMRHALTLAKRARDEREVPVGAVLVLNNRVIGEGWNRAIGLHDPTAHAEIMALRQGGLVMQNYRLTDATLYVTFEPCVMCAGAMIHSRIGRVVFGVRNSKRGAAGSLMNVLNYPGMNHCVEITEGILVDECAALLCDFYRMPRQVLNAQKKAQSSISSGGSSGGSSGSETPGASGSVTPKSSGGSSAGSTKDTITKTLKLRIVRPYNSAEVEKIVADEKNNREKIALEKNKDKVKEACSKHLKVAAYCTTQVERNACLFCKARKLDDKFYQKLRGQFPDAVFWQEIGEIFRQLQKQAAEIYNQSLIELYYEIFIKGKGFANASSVEHYLSDVCYTRAAELFKNAAIASGLRGKVKSNFRLKELKNMKSGLPTTKSDNFPIPLVKQKGGQYTGFEIGSHNDDFIIKIPFGRWQVKEEIDKYRPWEKFDFEQVRKNPKPISLLLSTQRRKRNKGWSKDEGTEAEIRKVMNGDYQTSYIEVKRGSKIGEKSAWMLNLSIDVPKIDKGVDPSIIGGIDVGVKSPLVCAINNAFSRYSISDNDLFRFNKKMFARRRILLKKNRHKRAGHGAKNKLKPITILTEKSRRFRKKLIERWACEIADFFIKNKVGTVQMESLESMKRKEDSYFNIRLRGFWPYAEMQNKIEFKLKQYGIEIRKVAPNNTSKTCSKCGHLNSYFNFEYRKKNKFPHFKCEKCYFKEDADYNAALNISNPRLKSTKEEP

SEQ ID NO: 1038 - protein, 726 aa, synthetic construct
SEVEFSHEYWMRHALTLAKRARDEREVPVGAVLVLNNRVIGEGWNRAIGLHDPTAHAEIMALRQGGLAMRNYRLVDATLYVTFEPCVLCAGAMVHSRIGRVVFGVRNSKRGAAGSLMNVLNHPGMNHRVEITGGILADECAALLCDFYRMPRQVFNAQKKARSNINSGGSSGGSSGSETLGTSESATPESSGGSSGGSAKNTITKTLKLRIVRPYNSAEVEKIVADEKNSREKIALERNKDKVKEACSEHLKVAAYCTTQVERNACLFCKARKLDDRFYQKLRGQFPDAVFWQETGEIFRQLQRQAAEIYNQSLIELYYEIFIRGKGFANASSVEHYLSDVCYTRAAELFKNAAIASGLRGKVKSNFRLKELKNMKSGLPTTKSDNFPIPLVKQKGGQYTGFEISSHNDDFIIKIPFGRWQVRKEIDKYRPWEKFDFEQVRKSPKPISLLLSTQRRKRNKGWSKDEGTEAEIRKVMNGDYQTSYIEVKRGSKIGEKSAWMLSLSIDVPKIDKGVDPSIIGGIDVGVKSPLVCAINNAFCRYSISDNDLFHFNKKMFARRRILLKKSRHKRAGHGAKNKLKPISILTEKSKRFRKKLIERWACEIADFFIKNKVGTVQMENLESMKRKEDSYFNIRLRGFWPYAEMQNKIEFKLKQYGIEIRKVAPNNTSKTCSKCGHLNNYFNFEYRKKNRFPHFKCEKCNFKENADYNAALNISNPKLKSTKEEP

SEQ ID NO: 1039 - protein, 726 aa, synthetic construct
SEVEFSHEYWMRHALTLAKRARDEREVPVGAVLVLNNRVIGEGWNRAIGLHDPTAHAEIMALRQGGLVMQNYRLIDATLYVTFEPCVMCAGAMVHSRIGRVVFGVRNSKRGAAGSLMNVLNYPGMDHRVEITGGILADECAALLCDFYRMPRRVFNAQRKAHSSINSGGSSGGSSGSVTPGTSESATPESSGGGFGDSAKNTITKTLQLRIVRPYNSAEVEKIVADEKNNREKIALEKNKDKVKEACSKHLKVASYCTTQVERNACLFCKARKLDDKFYQKLRGQFPDAVFWQELGEIFRQLQKQAAEIYNQSLIELYYEIFIKGKGLANASSVEHYLSDVCYTRAAELFKNAAIASGLRGKVKSNFKLKELKSMKSGLPSTKSDNFPIPLVKQKGGQYTGFEISSHNNDLIIKIPFGRWQVKREIDKYRPWEKFDFEQVRKSPKPISLLLSTQRRKRNKGWSKDEGTEAEIRKVMNGDYQTSYIEVKRGSKFGEKSAWMLNLSIDVPKIDKGVDPSIIGGIDVGVKSPLVCAINNAFSRYSISDNDLFRFNKKMFARRRILLGKNRHKRAGHGVKNKLKPITILTEKSGRFRKKLIERWACEIADFFVKNKVGTVQMENLESMKRKEDSYFNIRLRGFWPYAEMQNKIEFKLKQYGIKVRKVAPNNTSKTCSKCGHLNNYFSFEYRKKNKFPHFKCEKCNFKENADYNAALNISNPKLKSTKEEP

SEQ ID NO: 1040 - protein, 726 aa, synthetic construct
SEVEFSHEYWMHHALTLAKRARDEREVPVGAVLVLNNRVIGVGWNRAIGLHDPTAHAEIMALRQGGLVTQNYRLINATLYVTFEPCVMCAGAMIHSRIGRVVFGVRNSKHGAAGSLVNVLNYPGMNHRVEITEGILADECAALLCDFYRMPRQVFNARKKAQSSINSGGSSGGSSGSETPGTSESATPKSSGGSSGGSAKNTITKALKLRIVRPYNSAEVEKIVADEKNSREKIALEKNKDKVKEACSKHLKVAAYCTTRVERNACLFCKARKLDDKFYQKLRGQFPDAVFWQEIGEVFRQLQKQAAEIYNQSLIELYYEIFIKGKGFANASSVEHYLSDVCYTRAAELFKNAAIASGLRGKVKSNFRLKELKNMKSGLPTTKSDNFPIPLVKQKGGQYTGFEISSHNDDFIIKIPFGRWQVKKEIDKYRPWEKFDFEQVRKSPKPISLLLSTQRRKRNKGWSKDEGTEAEIRKVMSGDYQTSYIEVKRGSKTGEKSAWMLNLSIDVPKIDKGVDPSIIGGIDVGVKSPLVCAINNAFSRYSISDNDLFRFNKKMFARRRILLKKNRHKRAGHGAKNKLKPISILTGKSERFRKKLIERWACEIADFFIKNKVGTVQMENLESMKRREDSYFNIRLRGFWPYAEMQNKIEFKLKQYGIEIRKVAPNNTSKTCSKCGHLNNYFNFEYRRKNKFPHFKCERCNFKENADYNAALNISNPKLKSTKGEP

SEQ ID NO: 1041 - protein, 726 aa, synthetic construct
SEVEFSHEYWMRHALTLARRARDEREVPVGAILVLNNRVIGEGWNRAIGLHDPTAHAEIMALRQGGLVMQSYRLADATLYVTFEPCVMCAGAMIHSRIGRVVFGVRNSKHGAAGSLMNVLNYPGMNHRVEITEGILADECAALLCDFYRMPRRVFNAQKKAQSSINPGGSSGGSSGSETPGVSESVTPKSSGGSSGGSAKNTITKTLKLRIVRPYNSAEVEKIVADEKNNREKIALEKNKGKVKEACSKHLEVAAYCTTQVERNACLFCKARKLDDKFYQKLRDQFPDAVFWQELGEIFRQLQKQAAEIYNQSLIELYYEIFIKGKGFANASNVEHYLSDVCYTRAAELFKNAAIASGLRGKVKSNFRLKELKNMKSGLPTTKSDNFPIPLVKQKGGQYTGFEISSHNDDLIVKIPFGRWQVKKEIDKYRPWEKFDFEQVRKSPKPISLLLSTQRRKRNKGWSKDEGTEAEIRRVMNGDYQTSYIEVKRGSKIGEKSAWMLNLSIDVPKIDKGVDPSIIGGIDVGVKSPLVCAINNAFSRYSISDNDLFHFNKKMFARRRILLKKNRHKRAGHGAKNKLKPISILTGKSERFRKKLIERWACEIADFFIKNKVGTVQMENLESMKRKEDSYFNIRLRGFWPYAEMQNKIEFKLKQYGIEIRKVAPNNTSKTCSKCGHLNNYFNFEYRKKNKFPHFKCEKCNFKENADYNAALNISNPKLKGTKEKP

SEQ ID NO: 1042 - protein, 726 aa, synthetic construct
SEVEFSHEYWMRHALTLAKRARDEREVPVGAVLVLNNRVIGEGWNRTTGLHDPTAHAEIMALRQGGLVMRNYRLTDATLYVTFEPCVMCAGAMIHSRIGRVVFGVRNNKRGAAGSLMNVLNYPGMNHCVEITEGILVDECAALLCDFYRMPRQVLNAQKRAQSSISPGGSSGGSSGSETPGASESVTPKSSGGSSGGSAKNTVTKTLKLRIVRPYNSAEVEKIVADEKNNREKIALEKNKGKVKEACSKHLEVAAYCTTQVERNACLFCKARKLDDKFYQKLRGQFPDAVFWQELGEIFRQLQKQAAEVYNQSLIELYYEIFIKGKGFANASSVEHYLSDVCYTRAAELFKNAAIASGLRGKVKGNFRLKELKNMKSGLPTTKSDNFPIPLVKQKGGQYTGFEICNHNGDFIIKIPFGRWQVKQEIDKYRPWEKFDFGQVRKSPKPISLLLSTQRRKRNKGWSRDEGTEAEIRKVMNGDYQSSYIEVKRGSKIGEKSAWMLNLSIDVPKIDKGVDPSIIGGIDVGVRSPLVCAIDNAFSRYSISDNDLFHFNKKMFARRRILLKKNRHKRAGHGAKNKLKPLTILTRKSERFRKKLIERWACEVADFFIKNKVGTVQMENLESMKRREDSYFNIRLRGFWPYAEMQNKIEFKLRQYGIEIRKVAPNNTSKTCSKCGHLNNYFNFEFRKKNKFPHFKCEKCNFKEDADYNAALNISNPKLKSTKEEP

SEQ ID NO: 1043 - protein, 726 aa, synthetic construct
SEVEFSHEYWMRHALTLAERARDEREVPVGAVLVLNNRVIGEGWNRAIGLHDPTAHAEIMALRQGGLVMQNYRLTDATLYVTFEPCVMCAGAMIHSRIGRVVFGVRNSKRGAAGSLMNVLNYPGMNHCVEITEGILVDECAALLCDFYRMPRQVLNAQKKAQSSISSGGSSGGSSGSVTPGASGSVTPKSSGGSSAGSTKDTITKTLKLRIVRPYNSAEVEKIVADEKNNREEIALEKNKDKVKEACSKHLKVASYCTTQVERNACPFCKARKLDDKFYQRLRGQFPDAVFWQELGEILWQLQKQAAEVYNQSLVELYYEILIKGKGIANASSVEHYLSDVCYTRAAELFKNAAIASGLRNKIKSNFRLKELRNMKSGLPTTKSDNFPIPLVRQKGGQYTGFEISNHDGDFIIKIPFGRWQVKKEINKHRPWEKFDFEQVRKSPKPISLLLSTQRRRRNKGWSRDEGTEAEIRKVMNGDYQTSYIEVKRGSKIGEKGAWMLNLSIDVPKIDKGVDPSIIGGIDVGVKSPLVCAINNALSRYSISDNDLFHFNKKMFARRRILLKKNRHKRAGHGVKNKLKPISILTEKSKRFRKKLIERWACEIADFFIKNKVGTVQMENLESMKRKEDSYFNIRLRGFWPYAEMQNKIEFKLKQYGIEIRKVAPNNTSKTCSKCGHLNNYFNFEYRRMNKFPHFKCEKCNFKENADYNAALNISNPKLKSTKEEP

SEQ ID NO: 1044 - protein, 726 aa, synthetic construct
SEVEFSHEYWMRHALALAKRARDEREVPVGAILVLNNRVIGEGWNRAIGLHDPTAHAEIMALRQGGLVMQNYRLINATLYVTFEPCVMCAGAMIHSRIGRVVFGVRNSKHGAAGSLMNVLNYPGMNHRVEITEGILADECAALLCDFYRMPRQVFSARKKAQSSINSGGSSGGNSGSETPGTSESATPRSSGGSSGGSARNTITKTLKLRIVRPYNSAEVEKIVADEKNNRERIALEKNKDKVKEACSKHLKVAAYCTTQVERNACLFCKARRLDDKFYQKLRGQFPDAVFWQEIGEIFRQLQKQAAEIYNQSLVELYYEIFIKGKGIANASSVEHYLSDVCYTRAAELFRNAAIASGLRNKIKSNFRLKELRNMRSGLPTTKSDNFPIPLVRQKGGQYTGFEISNHDGDFIIKIPFGRWQVKKEINKHRPWEKFDFEQVRKSPKPISLLLSTQRRKRNKGWSKDEGTEAEIRKVMNGDYQTSYIEVKRGSKIGEKSAWMLNLSIDVPKIDKGVDPSIIGGIDVGVKSPLVCAINNSSSRYSICDNDLFRFNKKMFARRRILLKKNRHKRAGHGAKNKLKPITILTKKSERFRKKLIERWVCEVADFFIKNKVGTVQMENLESMKRKEDSYFNIRLRGFWPYAEMQNRIELKLKQYGIEIRRVAPNNTSRTCSKCGHLNNYFSFEYRKKSKFPHFKCEKCNFREDADYNAALNISNPKLKSTKEEP

SEQ ID NO: 1045 - protein, 726 aa, synthetic construct
SEVEFSHEYWMRHALTLAKRARDEREVPVGAVLVLNNRVIGEGWNRAIGLHDPTAHAEIMALRQGGLVMQNYRLTDATLYVTFEPCVMCAGAMIHSRIGRVVFGVRNSKRGAAGSLMNVLNYPGMNHCVGITEGILVDECAALLCDFYRMPRQVLNAQKKAQSSISSGGSSGGSSGSETPGASESATPKSSGGSSASSTKDTITKTLKLRIVRPYNSAEVEKIVADEKNNRERIALEKNKDKVKEACSKHLKVAAYCTTQVERNACLFCKARKLDDKFYQKLRGQFPDAVFWQEIGEIFRQLQKQAAETYNQSLIELYYEIFIKGKGVANANNVEHYLSDVCYTRAAELFKNAAIASGLRNKIKSNFRLKELRNMRSGLPTTKSDNFPIPLVKQKGGQYTGFEISSHNDDFIIKIPFGRWQAKKEIDKYRPWEKFDFEQVRKSPKPISLLLSTQRRRRNRGWSRDEGTEAEIRKVMNGDYQTSYIEVKRGSKIGAKSAWMLNLSIDVPKIDKGVDPSIIGGIDVGVKSPLVCAINNAFSRYSISDNDLFRFNKKMFARRRILLGKNRHKRAGHGVKNKLKPITILTEKSGRFRKKLIERWACEIADFFVKNKVGTVQMENLESLKRKEDSYFNIRLRGFWPYAEMQNKIEFKLKQYGIKVRKVAPNNTSKTCSKCGHLNNYFNFEYRKKNKFPHFRCEKCNFKENADYNAALNISNPKLKSAKEEP

SEQ ID NO: 1046 - protein, 726 aa, synthetic construct
SEVEFSHEYWMRHALTLAKRARDEREVPVGAVLVLNNRVIGEGWNRAIGLHDPTAHAEIMALRQGGLVMQNYRLIDATLYVTFEPCVMCAGAMIHSRIGRVVFGVRNSKHGAAGSLMNVLNYPGMNHRVEITEGILADECAALLCDFYRMPRQVFNARKKAQSSINPGGPSGGSSGSETPDTSESATPESSGGNSGGSAKDTITKTLKLRIVRPYNSAEVEKVVADEKNNREKIAIEKNKDKVKEACSKHLKVASYCTTQVERNACLFCKARKLDDKFYQGLRGQFPDAVFWQELGEIFRQLQKQAAEIYNQSLIELYYEILIKGKGIANASSVEHYLSDVCYTRAAELFKNAAIASGLRNKIKSNFRLKELRNMRSGLPTTKSDNFPIPLVRQKGGQYTGFEISNHDGDFIIKIPFGRWQVKKEINKHRPWEKFDFEQVRKSPKPISLLLSTQRRKRNKGWSKDEGTEAEIRKVMNGDYQTSYIEVKRGSKIGEKSAWMLNLSIDVPKIDKGVDPSIIGGIDVGVKSPLVCAINNAFSRYSISDNELFHFNKKMFARRRILLKKNRHKRAGHGAKNKLKPISILTEKSERFRKKLIEKWACEIADFFIKNKVGTVQMENLESMKRKEDSYFNIRLRGFWPYAEMQNKIEFKLKQYGIKVRKVAPNNTSKTCSKCGHLNNYFSFEYRKKNKFPHFKCEKCNFKENADYNAALNISNPKLKSTKEEP

SEQ ID NO: 1047 - protein, 726 aa, synthetic construct
SDVEFSHEYWMRHALTLAKRARDEREVPVGAVLVLNNHVIGEGWNRAIGLHDPTAHAEIMALRQGGLVMQNYRLTDATLYVTFEPCVMCAGAMIHSRIGRVVFGVRNSRRGAAGSLMNVLNYPGMNHCVEITEGILVDECAALLCDFYRMPRQVLNAQKKARSSISPGGSSGGSSGSETPGASGSVTPKSSGGSSAGSTKDTITKTLKLRIVRPYNSAEVEKIVADEKNSREKIALEKYKDKVKEACSKHLKVAAYCTTQVERNACLFCKARKLDDKFYQKLRGQFPDAVFWQETGEIFRQLQRQAAEIYNQSLIELYYEIFIKGKGFANASSVEHYLSDVCYTRAAELFKNAAIASGLRGKVKGNFRLKELKNMKSGLPTTKSDNFPIPLVKQKGGQYTGFEISSHNDDFIIKIPFGRWQAKKEIDKYRPWEKFDFEQVRKSPKPISLLLSTQRRKRNKGWSKDEGTEAEIRKVMYGDYQTSYIEVKRGSKIGEKSAWMLNLSIDVPKIDKGVDPSIIGGIDVGVKSPLVCAINNAFSRYSISDNDLFHFNKKVFARRRILLKKNRHRRAGHGAKNKLKPITILTEKSKRFRKKLIERWACEIADFFVKNKVGTVQMENLESMKRKEDSYFNIRLRGFWPYAEMQNKIEFKLKQYGIKIRKVAPNNTSRTCSECGHLNNYFSFEYRKKNKFPHFKCEKCNFKEDADYNAALNISNPKLKGTKEEL

SEQ ID NO: 1048 - protein, 726 aa, synthetic construct
SEVEFSHEYWMRHALTLAERARDEREVPVGAVLVLNNRIIGEGWNRAIGLHDPTAHAEIMALRQGGLVMQNYRLIDATLYVTFEPCVMCAGAMIHSRIGRVVFGVRNSKHGAAGSLVNVLNYPGMNHRVEITEGILADECAALLCDFYRMPRRVFNARMKAQSSISPGGSSGGSSGSETPSTSESATPESSGGSSGGSAKNTITKTLQLRIVRPYNSAEVEKIVADEKNNREKVALEKNKDKVREACSKHLKVASYCTTQVERNACPFCKARKLDDKFYQKLRGQFPDAVFWQELGEILRQLQKQAAEIYNQSLIELYYEIFIKGKGFANASSVEHYLSDVCYTRAAELFKNAAIASGLRGKVKSNFRLKELKNMKSGLPTTKSDNFPIPLVKQKGGQYTGFEISSHNDDFIIKIPFGRWQVKKEIDKYRPWEKFDFEQVRKSPKPISLLLSTQRRKRNKGWSKDEGTEAEIRKVMNGDYQTSYIEVKRGSKTGEKSAWMLNLSIDVPKIDKGVDPSIIGGIDVGVKSPLVCAINNAFSRYSISDNELFHFNKKMFARRRILLKKNRHKRAGHGAKNKLKPISVLTEKSGRFRKKLIERWACEIADFFIKNKVGTVQMENLGSMKRKEDSYFNIRLRGFWPYAEMQNKIEFKLKQYGIKIRKVAPNNTSKTCSKCGHLNNYFSFEYRKKNKFPHFKCEKCNFKEDADYNAALNISNPKLKSTKEEP

SEQ ID NO: 1049 - protein, 726 aa, synthetic construct
SEVEFSHEYWMRHALTLAKRARDEREVPVGAVLVLNNRVIGEGWNRAIGLHDPTAHAEIMALRQGGLVTQNYRLIDATLYVTFEPCVMCAGAMIHSRIGRVVFGVRNSKHGAAGSLVNVLNYPGMNHRVEITEGILADECAALLCDFYRMPRQVFNGRKKAQSSINSGGSSGGSSGSEAPGTSESATPESSGGSSGGSAKNTITKTLQLRIVRPYNSAEVEKIVADEKNSREKIALERNKDKVKEACSEHLKVAAYCTTQVERNACLFCKARKLDDRFYRKLRGQFPDAVFWQETGEIFRQLQRQAAEIYNQSLIELYYEIFIKGKGFANASSVEHYLSDVCYTRAAELFKNAAIASGLRGKVKSNFRLKELKNMKSGLPTTKSDNFPIPLVKQKGGQYTGFEISSLNDDFIIKIPFGRWQVKKEIDKYRPWEKFDFEQVRKSPKPISLLLSTQRRKRNKGWSKDEGTEAEIRKVMNGDYQTSYIEVKRGSKIGEKSAWMLSLSIDVPKIDKGVDPSIVGGIDVGVKSPLVCAVNNALGRYSISDNDLFHFNKKMFARRRILLRKNRHKRAGHGARNKLKPITVLTEKSERFRKKLIERWACEIANFFIKNKVGTVQMENLESMKRKEDSYFNIRLRGFWPYAEMQNKIEFKLKQYGIEIRKVAPNNTSKTCSKCGHLNNYFNFEYRRKNKFPYFKCEKCNFKENADYNAALNISNPKLKSTKEEP

SEQ ID NO: 1050 - protein, 726 aa, synthetic construct
SEVEFSHEYWMRHALTLAKRARDEREVPVGAVLVLNNRVIGGGWNRAIGLHDPTAHAEIMALRQGGLVMQSCRLVDATLYVTFEPCVMCAGAMIHSRIGRVVFGVRNSKHGAAGSLMNVLNYPGMNHRVEITEGILADECAALLCDFYRMPHRVFNGRKKAQSSINPGGSSGGSSGSETPGTSESATPESSGGSSGSSAKNTITKTLKLRIVRPYNSAEVEKIVADEKNNREKIALEKNKDKVKEACSKHLKVAAYCTTQVERNACLFCKARRLDDKFYQKLRGQFPDAVFWQELGEILRQLQKQAAEIYNQSLIELYYEIFIKGRGFANASSVEHYLSDVCYTRAAELFKNAAIASGLRGKVKSNFRLKELKNMKSGLPTTKSDNFPIPLVKQKGGQYTGFEISSHNDDFIIKIPFGRWQVKKEINKFRPWEKFDFEQVRKSPKPISLLLSTQRRKRNKGWSRDEGTEAEIRKVMNGDYQTSYIEVKRGSKIGEKSAWMLNLSIDVPKIDKGVDPSIIGGIDVGVKSPLVCAINNAFSRYSISDNDLYRFNKKMFARRRILLKKSKHKRAGHGAKNKLKPITILTEKSGRFRKKLIERWACEIADFFIKNKVGTVQMENLEGMKRKEDSYFNIRLRGFWPYAEMQNRIEFKLKQYGIEIRKVAPNNTSKTCSKCGHLNNYFNFEYRKKNKFPHFKCEKCNFKENADYNAALNISNPKLKGTKEEP

SEQ ID NO: 1051 - protein, 726 aa, synthetic construct
SEVEFSHEYWMRHALTLAKRARDEREVPVGAILVLNNRVIGEGWNRAIGLHDPTAHAEIMALRQGGLVMQNYRLIDATLYVTFEPCVMCAGAMIHSRIGRVVFGVRNSKHGAAGSLVNVLNYPGMNHRVEITEGILADECAALLSDFYRMPRRVFNAQKKAQSSINSGGSSGGGSGSETPSTSESTTPESSGGGPSGSTKNTITKTLKLRIVRPYNSAEVEKIVADEKNNREKIALEKNKDKVREACSKHLKVASYCTTQVERNACPFCKARKLDDKFYQKLRGQFPDAVFWQELGEILRQLQKQAAEIYNQSLIELYYEIFIKGRGFANASSVEHYLSDVCYTRAAELFKNAAIASGLRGKVKGNFRLKELKNMKSGLPTTKSDNFPIPLVKQKGGQYTGFEISGHNDDFIIKIPFGRWQAKKEIDKYRPWEKFDFEQVRKSPKPISLLLSTQRRKRNRGWSKDEGTEAEIRKVMNGDYQTSYIEVKRGSKIGEKSAWMLNLSIDVPKIDKGVDPSIIGGIDVGVKSPLVCAINNAFSRYSISDNDLFRFNKKMFARRRILLGKNRHKRAGHGVKNKLKPITILTEKSGRFRKKLIERWACEIADFFIRNKVGTVQMENLEGMKRKEDSYFNIRLRGFWPYAEMQNKIEFKLKQYGIEIRKVAPNNTSKTCSRCGHLNNYFSFEYRKKNKFPHFKCEKCNFKENADYNAALNISNPKLRSTKEEP

SEQ ID NO: 1052 - protein, 726 aa, synthetic construct
SEVEFSHEYWMRRALTLAKRARDEREVPVGAVLVLNNRVIGVGWNRAVGLHDPTAHAEIMALRQGGLVMQNYRLIEATLYVTFEPCIMCAGAMIHSRIGRVVFGVRNSKRGAAGSLMNVLNYPGMNHRVEVTEGILADECAALLCDYYRMPRQVFNARKKAQSSTNSGGSSDGGSGSETPSTSESATPGSSGGSSGGSAKNTITKTLKLRIVRPYNSAEVEKIVADEKNNREKIALEKNKDKVKEACSEHLKVAAYCTTQVERNACLFCKARKLDDKFYQKLRGQFPDAVFWQEIGEIFRQLQRQAAEIYNQSLIELYYEIFIKGKGFANASNVEHYLSDVCYTRAAELFKNAAIASGLRGKVKSNFRLKELKNMKSGLPTTKSDNFPIPLVKQKGGQYTGFEISSRNDDFIIKIPFGRWQAKKEIDKYRPWEKFDFEQVRRSPKPISLLLSTQRRKRNRGWSKDEGTEAEIRKVMNGDYQTSYIEVKRGSKIGEKSAWMLNLSIDVPKIDKGVDPSIIGGIDVGVKSPLVCAINNAFSRYSISDNDLFHFNKKVFARRRILLKKNRHRRAGHGAKNKLKPITILTEKSKRFRKKLIERWACEIADFFIKNKVGTVQMENLESMKRKEDSYFNIRLRGFWPYAEMQNKIEFKLKQYGIKIRKVAPNNTSRTCSKCGHLNNYFSYEYRKKNKFPHFKCEKCNFKEDADYNAALNISNPKLKGTKEEL

SEQ ID NO: 1053 - protein, 726 aa, synthetic construct
SEVEFSHEYWMRHALTLAKRARDEREVPVGAVLVLNNRAIGEGWNRAIGLHDPTAHAEIMALRQGGLVMQNYRLTDATLYVTFEPCVMCAGAMIHSRIGRVVFGVRNSKRGAAGSLMNVLNYPGMNHCVEITEGILVDECAALLCDFYRMPRQVLNAQKRAQSSISPGDSSGGSSGSETPGASGSVTPKSSGGSSAGSTKDTITKTLKLRIVRPYNSAEVEKIVADEKNSREKIALEKNKDKVKEACSKHLKVASYCTTQVERNACLFCKARKLDDKFYQKLRGQFPDAVFWQEVGGIFRQLQRQAAEIYNQSLIELYYEIFIKGKGFANASSVEHYLSDVCYTRAAELFKNAAIASGLRGKVKSNFRLKELKNMKSGLPTTKSDNFPIPLVKQKGGQYTGFEISNHNSDFIIKIPFGRWQVKKEINKYRPWEKFDFEQVRKSPKPISLLLSTQRRKRNKGWGKDEGTEAEIRKVMNGDYQTSYIEVKRGSKIGEKSAWMLSLSIDVPKIDKGVDPSIIGGIDVGVKSPLVCAINNALNRYSISDNDLFHFNKKMFARRRILLKKNRHRRAGHGAKNKLKPITVLTEKGKRFRKKLIERWACEIANFFIKNKVGTVQMENLESMKRKEDSYFNIRLRGLWPYAEMQNKIEFKLKQYGIGVRKVAPNNTSKTCSKCGHLNNYFNFEYRKKNKFPRFKCEKCNFKENADYNAALNISNPKLKSTKEEP

SEQ ID NO: 1054 - protein, 726 aa, synthetic construct
SEVEFSHEYWMRHALALAKRARDEREVPVGAVLVLNNRVIGEGWNRAIGLHDPTAHAEIMALRQGGLVMQNYRLTDATLYVTFEPCVMCAGAMVHSRIGRVVFGVRNSKRGAAGSLMNVLNYPGVNHCVEITEGILVDECAALLCDFYRMPRQVLNAQKKAQSSISSGGSSGGCSGSEMPGASESVTPESSGGSSAGSTKNTITKTLKLRIVRPYNSAEVEKIVADEKNSREKIALERNKDKVKEACSEHLKVAAYCTTQVERNACLFCKARKLDDKFYQKLRGQFPDAVFWQEIGEIFRQLQKQAAEIYNQSLIELYYEIFIKGKGFANASSVEHYLSDVCYTRAAELFKNAAIASGLRGKVKSNFRLKELKNMKSGLPTTKSDNFPIPLVKQKGGQYTGFEISSHNDDFIIKIPFGRWQVKKEIDKYRPWEKFDFEQVRKSPKPISLLLSTQRRKRNKGWGKDEGTEAEIRKVMNGDYQTSYIEVKRGSKIGEKSAWMLNLSIDVPKIDKGVDPSIIGGIDVGVKSPLVCAINNAFSRYSISDNDLFHYNKKMFARRRILLKKNRHKRAGHGAKNKLKPISILTEKNKRFRKKLIERWACEIADFFIKNKVGTVQIENLESMKRKEDSYFNIRLRGLWPYAEMQNKIEFKLKQYGIEIRKVAPNNTSKTCSKCGHLNNYFNFEYRKKNKFPHFKCEKCNFKENADYNAALNISNPKLKSTKEES

SEQ ID NO: 1055 - protein, 726 aa, synthetic construct
SEVEFSHEYWMRHALTLAKRARDEREVPVGAILVLNNRVIGEGWNRAIGLHDPTAHAEIMALRQGGLVMQNYRLTGATLYVTFEPCVMCAGAMIHSRIGRVVFGVRNSKRGAAGSLMNVLNYPDMNHCVEITEGILADECAALLCDYYRMPRQVFNARKKVQSSINSGGSSGGSGGSKTPGTSESATPESPGGSSGGSAKNTITKTLKLRIVRPYNSAEVEKIVADEKNNREKIALEKNKDKVREACSKHLKVAAYCTTQVERNACLFCKARRLDDKFYQKLRGQFPDAVFWQEIGEIFRQLQKQAAEIYNQSLIELYYEIFVKGKGIANASRVEHYLSDVCYTRAAELFKNAAIASGLRNKIKSNFRLKELRNMKSGLPTTKSDNFPIPLVKQKGGQYTGFEISCHNDDFVIKIPFGRWQVKKEIDKYRPWEKFDFEQVRKSPKPISLLLSTQRRKRNRGWSKDEGTEAEVKKVMNGDYQISYIEVKRGSKIGEKSAWTLNLSIDVPKIDKGVDPSIIGGIDVGVKSPLVCAINNAFSRYSISDNDLFHFNKKMFARRRILLKKSKHKRAGHGAKNKLKPISILTEKSKRFRKKLIERWACEIADFFVKNKVGTVQMEDLESMKRRGDSYFNIRLRGFWPYAEMQNKIEFKLKQYGIVVRKVAPNNTSKTCSQCGHLNNYFNFEYRKKNKFPYFKCEKCNFKENADYNAALNISNPQLKSTKGEP

SEQ ID NO: 1056 - protein, 726 aa, synthetic construct
SEVEFSHEYWMRHALTLAKRARDEREVPVGAVLVLNNRVIGEGWNRAIGLHDPTAHAEIMALRQGGLVMQNYRLIDATLYVTFEPCVMCAGAMIHSRIGRVVFGVRNNKHGAAGSLVNVLNYPGMNHRVEITEGILANECAALLCDFYRMPRQVFNARKKAQSSINPGGSSGGSSGSETPGTSESATPESSGGSSGGSAKNTITKALKLRIVRPYNSAEVEKIVADEKNNREKIALEKNKDKVKEACSKHLKVAAYCTTQVERNACPFCKARRLDDKFYQKLRGQFPDAVFWQELGEIFRQLQKQAAEIYNQSLIELYYEIFVKGKGFANASSVEHYLSDVCYTRAAELFKNAAIASGLRGKVKSNFRLKELRNMKSGLPTTKSDNFPIPLVKQKGGQYTGFEISSHNDDFIIKIPFGRWQVKKGIDKYRPWEKFDFEQVRKSPKPISLLLSTQRRKRNKGWSKDEGTEAEIRKVMNGDYQTSYIEVKRGSKIGEKSAWMLNLSIDVPKIDKGVDPSITGGIDVGVKSPLVCAINNALSRYSINDNDLFHFNKKMFARRRILLRKNRHKRAGHGARNKLKPITVLTEKSKRFRKKLIERWACEIANFFIKNKVGTVQMENLESMKRREDSYFNIRLRGFWPYAEMQNKIEFKLKQYGIEIRKVAPSNTSKTCSKCGHLNNYFNFEFRKKNKFPHFKCEKCNFKENADYNAALNISNPKLKSTKEEP

SEQ ID NO: 1057 - protein, 726 aa, synthetic construct
SEVEFSHEYWMRHALTLAKRARDEREVPVGAVLVLNNRVIGEGWNRTIGLHDPTAHAEIMALRQGGLVMQNYRLTDATLYVTFEPCVMCAGAMIHSRIGRVVFGVRNSKRGAAGSLMNVLNYPGMNHCVEITEGILVDECAALLCDFYRMPRQVLNAQKKAQSSISSGGSSGCSSGSETPGASESVTPKSSVGSSAGSTKNTITKTLKLRIVRPYNSAEVEKIVADEKDNRERIALEKNKDKVKEACSKHLMVASYCTTQVERSACLFCKARELDGRFYQKLRGQFPDAVFWQELGEVFRQLQKQAAEIYNQSLIELYYEIFIKGKGFANASSVEHYLSDVCYTRAAELFRNAAIASGLRGKVKSNFRLKELKNMKSGLPTTKSDNFPIPLVKQKGGQYTGFEISSHNDDFIIKIPFGRWQVKKEIDRYRPWEKFDFEQVRKSPKPISLLLSTQRRKRNKGWSKDEGTEAEIRKVMNGDYQTSYIEVKRGSKIGEKSAWMLNLSIDVPRIDKGVDPSIIGGIDVGVKSPLVCAINNALSRYSISDNDLFHFNKKMFARRRILLRKNRHKRAGHGAKNKLKPITILTEKSGRFRKKLIERWACEIADFFVKNKVGTVQMEDLESMKRKEDSYFNIRLRGFWPYAEMQNKIEFKLKQYGIKVRKVAPNNTSKTCSKCGHLNNYFSFEYRKKNKFPHFKCEKCNFKENADYNAALNISNPKLKSTKEEP

SEQ ID NO: 1058 - protein, 726 aa, synthetic construct
SEVEFSHEYWMRHALTLAKRARDEREVPVGAVLVLNNRVIGEGWNRAIGLHDPTAHAEIMALRQGGLVMQNHRLVDATLYVTFEPCVMCAGAMVHSRVGRVVFGVRNSKRGAAGSLMNVLDYPGMGHRVEITEGILADECAALLCDFYCMPRQVFNAQKRAQSSINSGGSSGGSSGSETPGTSESATPESSGGGSSGSAKNTITKTLQLRIVRPYNSAEVEKIVADEKNNREKIALEKNKDKVREACSKHLKVASYCTTQVERNACPFCKARKLDDKFYQKLRGQFPDAVFWQELGEVLRQLQKQAAEIYNQSLIELYYEIFIKGKGIASASRVGHYLSDVCYTRAAELFKNAAIASGLRGKVKSNFRLKELKNMKSGLPTTKSDNFPIPLVKQKGGQYTGFEISSHNDDFIIKIPFGRWQVKKEIDKYRPWEKFDFEQVRKSPKPISLLLSTQRRKRNKGWSKDEGTEAEIRKVMNGDYQTSYIEVKRGSKTGEKSAWMLNLSIDVPKIDKGVDPSIIGGIDVGVKSPLVCAINNAFSRYSISDNDLFRFNKKMFARRRILLKKNRHKRAGHGVKNKLKPISILTGKSERFRKKLIERWACEIADFFIKNKVGTVQMENLESMKRKEDSYFNIRLRGFWPYAEMQNKIEFKLKQYGIEIRKVAPNNTSKTCSKCGHLNNYFNFEYRKKNKFPHFKCEKCNFKENADYNAALNISNPKLKSTKEEP

SEQ ID NO: 1059 - protein, 726 aa, synthetic construct
SEVEFSHEYWMRHALTLAKRARDEREVPVGAILVLNNRVIGEGWNRAIGLHDPTAHAEIMALRQGGLVMQNYRLIDATLYVTFEPCVMCAGAMIHSRIGRVVFGVRNSKHGAAGSLMNVLNYPGMNHRVEITEGILADECAALLCDFYRMPHQVFNARKKAQSSINPGGSSGGSSGSETPGTSESATPESSGGGSSGSAKNTITKTLQLRIVRPYNSAEVEKIVADEKNNREKIALEENKDKVREACNKHLKVASYCTTQVERNACPFCKARKLDDKFYQKLRGQFPDAVFWQELGEILRQLQKQAAEIYNQSLIELYYEIFIKGKGFANASSVEHYLSDVCYTRAAELFKNAAIASGLRGKVKSNFRLKELKNMKSGLPTTKSDNFPIPLVKQKGGQYTGFEISSHNDDFIIKIPFGRWQVKKEIDKYRPWEKFDFEQVRKSPKPISLLLSTQRRKRNKGWSKDEGTEAEIRKVMNGDYRTSYIEVKRGSRIGEKSAWMLNLSIDVPKIDKGVDPSIIGGIDVGVKSPLVCAINNAFSRYSISDNDLFHYNKKMFARRRILLKKNRHKRAGHGAKNKLKPISILTEKNKRFRKKLIERWACEIADFFIKNKVGTVQIENLESMKRKEDSYFNIRLRGFWPYAEMQNKIEFKLKQYGIEIRKVAPNNTSKTCSKCGHLNSYFNFEYRKKNKFPHFRCEKCNFRENADYNAALNISNPKLRSTKEEP

SEQ ID NO: 1060 - protein, 726 aa, synthetic construct
SEVEFSHEYWMRHALTLAKRARDEREVPVGAVLVLNNRVIGEGWNRAIGLHDPTAHAEIMALRQGGLVMQNYRLIDATLYVTFEPCVMCAGAMVHSRIGRVVFGVRNSKRGAAGSLMNVLDYPGMGHRVEITEGILADECAALLCDFYRMPRQVFNAQKRAQSSINSGGSSGGSSGSVTPGASESVTPKSSGGSSGGSAKNTITKTLKLRIVRPYNSAEVEKIVADEKNNREKIALEKNKGKVKEACSKHLEVAAYCTTQVERNACLFCKARKLDDKFYQKLRGQFPDAVFWQELGEIFRQLQKQAAEIYNQSLIELYYVIFIKGKGLANASSVEHYLSDVCYTRAAELFKNAAIASGLRGKVKSNFKLKELKSMKSGLPSTKSDNFPIPLVRQKGGQYTGFEISNHDGDFIIKIPFGRWQVKKEINKHRPWEKFDFEQVRKSPKPISLLLSTQRRKRNKGWSKDEGTEAEIRKVMNGDYQTSYIEVKRGSKIGEKSAWMLNLSIDVPKIDKGVDPSIIGGIDVGVKSPLVCAINNAFSRYSISDNDLFHFNKKMFARRRILLKKNRHKRAGHGAKNKLKPISILTEKSERFRKKLIERWACEIADFFIKNKVGTVQMENLESMKRREDSYFNTRLRGFWPYAEMQNKIEFKLKQYGIKIRKVAPNNTSKTCSKCGHLNNYFNFEYRKKNKFPHFKCEKCGFKENADYNAALNISNPKLKSTKEEP

SEQ ID NO: 1061 - protein, 726 aa, synthetic construct
SEVEFSHEYWMRHALTLAKRARDEREVPVGAILVLNNRVIGEGWNRAIGLHDPTAHAEIMALRQGGLAMQNYRLVDATLYVTFEPCVLCAGAMVHSRIGRVVFGVRNSKRGAAGSLMNVLNHPGMNHRVEITGGILADECAALLCDFYRMPRQVFNAQKKARSNINSGGSSGGSSGSETLGTSESATPESSGGSSGGSAKNTITKTLKLRIVRPYNSAEVEKIVADEKNNREKIALEKNKDKVKEACSEHLKVAAYCTTQVERNACLFCKARKLDDKFYQKLRGQFPDAVFWQELGEILRQLQKQAAEIYNQSLIELYYEIFIKGKGFANASSVEHYLSDVCYTRAAELFRNAAIASGLRGKVKSNFRLKELKNMKSGLPTTKSDNFPIPLVKQKGGQYTGFEISSHNDDFIIKIPFGRWQVKKEIDKYRPWEKFDFEQVRKSPKPISLLLSTQRRKRNKGWSKDEGTEAEIRKVMNGNYQTSFIEVKRGSKIGEKSAWMLSLSIDVPKIDKGVDPSIIGGIDVGVKSPLVCAINNAFSRYSISDNDLFRFNKKMFARRRILLKKNRHKRAGHGVKNKLKSISILTEKSKRFRKKLIERWACEIADFFIKNKVGTVQMENLESMKRKEDSYFNIRLRGFWPYAEMQNKIEFKLKQYGIEIRKVAPNNTSKTCSKCGHLNNYFNFEYRRKNKFPHFKCEKCNFKEDADYNAALNISNPKLKSTKEEP

SEQ ID NO: 1062 - protein, 726 aa, synthetic construct
SEVEFSHEYWMRHALTLAKRARDEREVPVGAVLVLNNRVIGEGWNRTTGLHDPTAHAEIMALRQGGLVMRNYRLTDATLYVTFEPCVMCAGAMIHSRIGRVVFGVRNSKRGAAGSLMNVLNYPGMNHCVEITEGILVDECAALLCDFYRMPRQVLNAQKKAQSSISPGGSSGGSSGSETPGASESVTLKSSGGSSGGSAKNTITKTLKLRIVRPYNSAEVEKIVADEKNNREKIALEKNKGKVKEACSRHLEVAAYCTTQVERNACLFCKARKLDDKFYQKLRGQFPDAVFWQELGEIFRQLQKQAAEIYNQSLIELYYEIFIKGKGFANASSVEHYLSDVCYTRAAELFKNAAIASGLRGKVKSNFRLKELKSMKSGLPTTKSDNFPIPLVKQKGGQYTGFEISSHNDDFIIKIPFGRWQVKEEIDKYRPWEKFDFEQVRKNPKPISLLLSTQRRKGNKGWSKDEGTEAEIRKVMNGDYQTSYIEVKRGSKIGEKSAWMLNLSIDVPKIDKGVDPSIIGGIDVGVKSPLVCAINNAFSRYSISDNDLFHFNKKMFARRRILLKKNRRRRAGHGAKNKLKPITILTEKSVRFRKKLIERWACEIADFFIKNKVGTVQMENLESMKRKEDSYFNIRLRGFWPYAEMQSKIEFKLKQYGIVVRKVAPNNTSKTCSKCGHLNNYFNFEYRKKNKFPHFKCEKCNFKEDADYNAALNISNPKLKSTKGEP

SEQ ID NO: 1063 - protein, 726 aa, synthetic construct
SEVEFSHEYWMRHALTLAKRARDEREVPVGAVLVLNNRVIGEGWNRAIGLHDPTAHAEIMALRQGGLAMQNYRLVDATLYVTFEPCVLCAGAMVHSRIGRVVFGVRNSKRGAAGSLMNVLNHPGMNHRVEITGGILADECAALLCDFYRMPRQVFNAQKKARSNINSGGSSGGSSGSETPGASESVTPKNSGGSSASSTKNTITKTLKLRIVRPYNSAEVEKIVADEKNSREKIALEKNKDKVKEACREHLKVAAYCTTQVERSACLFCKARKLDDRFYQKLRGQFPDAVFWQEISEIFRQLQKQAAEIYNQSLIELYYEVLIKGKGIANASRVEHYLSDVCYTRAAELFKNAAIASGLRSKIKSNFRLRELRNMKSGLPTTKSDNFPIPLVRQKGGQYTGFEISNHNGDFIIKIPFGRWQVKKEISKHRPWEKFDFEQVRKSPKPISLLLSTQRRKRNKGWGKDEGTEAEIRKVMNGDYQTSYIEVKRGSKIGEKSAWMLNLSIDVPKIDKGVDPSIIGGIDVGVKSPLVCAINNALSRYSISDNDLFHFNKKMFARRRILLRKNRHKRAGHGARNKLKPITVLTEKGERFRKKLIERWACEIANFFIKNKVGTVQMENLESMKRKEDSYFNIRLRGFWPYAEMQNKIEFKLKQYGIEIRRVAPNNTSRTCSKCGHLNNYFNFEYRRKNKFPHFKCEKCNFKEDADYNAALNISNPKLKSTKEEP

SEQ ID NO: 1064 - protein, 726 aa, synthetic construct
SEVEFSHEYWMRRALTLAKRARDEREVPVGAVLVLNNRVIGVGWNRAAGLHDPTAHAEIMALRQGGLVMQNYRLVEATLYVTFEPCIMCAGAMIHSRIGRVVFGVRNSKRGAAGSLMNVLNYPGMNHRVEITEGILADECAALLCDFYRMPRQVFNARKKARSNINSSGSSGGSSGSETPGTSESATPESSGGSSGGSAKNTITKTLKLRIVRPYNSAEVEKIVADEKNNREKIALEKNKDKVKEACSEHLKVAAYCTTQVERNACLFCKARKLDDKFYQKLRGQFPDAVFWQEISEIFRQLQKQAAEIYNQSLIELYYEIFIKGKGFANASSVEHYLSDVCYTRAAELFKNAAIASGLRGKVKSNFRLKELRNMRSGLPTTKSDNFPIPLVRQKGGQYTGFEISNHDGDFIIKIPFGRWQVKKEINKHRPWEKFDFEQVRRSPKPISLLLSTQRRKRNKGWSKDEGTEAEIRKVMNGDYQTSYIEVKRGSKIGEKSAWMLNLSIDVPKIDKGVDPSIIGGIDVGVKSPLVCAINNAFSRYSISDNDLFHFNKKMFARRRILLKKNRHKRAGHGAKNKLKPITILTEKSKRFRKKLIERWACEIADFFIKNKVGTVQMENLESMKRKEDSYFNIRLRGFWPYAEMQNKIEFKLKQYGIEIRKVAPNNTSRTCSKCGHLNGYFNFEYRKKNKFPHFKCEKCNFKENADYNAALNISNPKLKSTKEEP

SEQ ID NO: 1065 - protein, 726 aa, synthetic construct
SEVEFSHEYWMRHALTLAKRARDEREVPVGAVLVLNNRVIGEGWNRTTGLHDPTAHAEIMALRQGGLVMQNHRLVDATLYVTFEPCVLCAGAMVHSRIGRVVFGVRNSKRGAAGSLMNVLNYPGMNHRVEITEGILADECAALLCDFYRMPRQVFNARKKARSNINSSGSSGGSSGSETPGTSESATPESSGGSSGGSAKNTITKTLKLRIVRPYNSAEVEKIVADEKNNREKIALEKNKDKVKEACSEHLKVAAYCTTQVERNACLFCKARKLDDKFYQKLRGQFPDAVFWQEIGEIFRQLQKQAAEIYNQSLIELYYEIFIKGKGIANASSVEHYLSDVCYTRAAELFKNAAIASGLRGKVKSNFRLKELKNMKSGLPTTKSDNFPIPLVKQKGGQYTGFEISSHNDDFIIKIPFGRWQVKKEIDKYRPWEKFDFEQVRKSPKPISLLLSTQRRKRNKGWSKDEGTEAEIRKVMNGDYQTSYIEVKRGSKIGEKSAWMLNLSIDVPKIDKGVDPSIIGGIDVGVKSPLVCAINNALSRYSISDNDLFHFNKKMFARRRILLRKNRHKRAGHGAKNKLKPITIMTEKSKRFRKKLIEKWACEIADFFIKNKVGTVQMENLESMKRREDSYFNIRLRGFWPYAEMQNKIEFKLKQYGIGIRKVAPNNTSKTCSKCGHLNNYFNFEYRKKNKFPHFKCEKCNFKEDADYNAALNISNPKLKGTKEEL

SEQ ID NO: 1066 - protein, 726 aa, synthetic construct
SEVEFSHEYWMRHALTLAKRARDEREVPVGAVLVLNNRVIGEGWNRAIGLHDPTAHAEIMALRQGGLVMQNYRLIDATLYVTFEPCVMCAGAMVHSRIGRVVFGVRNSKRGAAGSLMNVLDYPGMGHRVEITEGILADECAALLCDFYCMPRQVFNAQKRAQSSINSGGSSGGSSGSETPGTSESATPGSSGGGSSGSAKNTITKTLQLRIVRPYNSAEVEKIVADEKSNREKIALEENKDKVKEACSKHLKVAAYCTTQVERNACLFCKARKLDDKFYQKLRGQFPDAVFWQELGEIFRQLQKQAAEIYNQSLIELYYVIFIKGKGLANASSVEHYLSDVCYTRAAELFKNAAIASGLRGKVKSNFKLKELKSMKSGLPTTKSDNFPIPLVKQKGGQYTGFEISSHNDDFIIKIPFGRWQVKKEIDKYRPWEKFDFEQVRKSPKPISLLLSTQRRKRNKGWSKDEGTEAEIRKVMNGDYQTSYIEVKRGSKIGEKSAWMLNLSIDVPKIDKGVDPSIIGGIDVGVKSPLVCAINNAFGRYSISDNDLFRFNKKMFARRRILLGKNRHKRAGHGVKNKLKPITILTEKSGRFRKKLIERWACEIADFFVKNKVGTVQMENLESMKRKEDSYFNIRLRGFWPYAEMQNKIEFKLKQYGIKVRKVAPNNTSKTCSKCGHLNNYFSFEYRKRNKFPHFKCEKCNFKENADYNAALNISNPKLKSTKEEP

SEQ ID NO: 1067 - protein, 726 aa, synthetic construct
SEVEFSHEYWMRHALTLAKRARDEREVPVGAILVLNNRVIGEGWNRAIGLHDPTAHAEIMALRQGGLVMQNYRLIDATLYVTFEPCVMCAGAMIHSRIGRVVFGVRNSKHGAAGSLVNVLNYPGMNHRVEITEGILVDECAALLCDFYRMPRQVLNAQKKAQSSISSGGSSGGSSGSETPGAGESVTPKSSVGSSAGSTKNTITKTLKLRIVRPYNSAEVERIVADEKNNREKIALEKNKDKVREACSKHLKVAAYCTTQVERNACLFCKARKLDDKFYQKLRGQFPDAVFWQEIGEIFRQLQKQAAEIYNQSLIELYYEIFIKGKGFANACSVEHYLSDVCYTRAAELFKNAAIASGLRGKVKSNFRLKELKNMKSGLPTTKSDNFPIPLVKQKGGQYTGFEISSHNDDFIIKIPFGRWQVKEEIDKYRPWEKFDFEQVRKNPKPISLLLSTQRRKRNKGWSKDEGTEAEIRKVMNGDYQTSYIEVKRGSKIGEKSAWMLNLSIDVPKIDKGVDPSIIGGIDVGVKSPLVCAINNAFSRYSISDNDLFRFNKKVFARRRILLKKNRHKRAGHGTKNKLKPITILAEKSGRFRKKLIERWACEIANFFIKNKVGTVQMENLEGMKRKEDSYFNIRLRGFWPYAEMQNKIEFKLKQYGIKIRKVAPNNTSKTCSKCGHLNNYFSFEYRKKNKFPHFKCEKCNFREDADYNAALNISNPKLRGAKEEL

SEQ ID NO: 1068 - protein, 726 aa, synthetic construct
SEVEFSHEYWMRHALTLAKRARDEREVPVGAVLVLNNRVIGEGWNRAIGQHDPTAHAEITALRQGGLVMQNYRLIDATLYVTFEPCVMCAGAMIHSRIGRVVFGVRNSKHGAAGSLVNVLNYPGMNHRVEITEGILADECAALLCDFYRMPRQVFNARKKAQPSINPGGSSGGSSGSETPGTSESATPESSGGSSGGSAKNTITKTLKLRIVRPYNSAEVEKIVADEKNNREKIALEKNKDKVKEACSKHLKVAAYCTTQVERNACLFCRARKLDDKFYQKLRGQFPDAVFWQEIGEIFRQLQKQAAEIYNQSLIELYYEIFIKGKGFANASSVEHYLSDVCYTRAAELFKNAAIASGLRGKVKSNFRLKELKNMKSGLPTTKSDNFPIPLVKQKGGQYTGFEISSHNDDFIIKIPFGRWQVKKEIDKYRPWEKFDFEQVRKSPRPISLLLSTQRRKRNKGWSKDEGTEAEIRKVMNGDYQTSYIEVKRGSKIGEKSAWMLSLSIDVPKIDKGVDPSIIGGIDVGVKSPLVCAINNAFSRYSISDNDLFHFNKKMFARRRILLKKNRHKRAGHGAKNKLKPITILTEKSRRFRKKLIERWACEIADFFIKNKVGTVQMENLESMKRREDSYFNIRLRGFWPYAEMQNKIEFKLKQYGIEIRKVAPYNTSKTCSKCGHLNNYFNFEYRKKNKFPHFKCEKCNFKENADYNAALNISNPKLKGTKEEP

SEQ ID NO: 1069 - protein, 726 aa, synthetic construct
SEVEFSHEYWMRHALTLAKRARDEREVPVGAVLVLNNRVIGEGWNRAIGLHDPTAHAEIMALRQGGLVLQNYRLVDATLYVTFEPCVLCAGAMVHSRIGRVVFGARNSKRGAAGSLMNILNYPGMNHRVEITEGILADECAALLCDFYRMPRQVFNAQKKAQSSINSGGSSGGSSGSETPSTSESPTPESPGGSSGGSAKNTITKTLKLRIVRPYNSAEVEKIVADEKNNREKIALEKNKDKVKEACSKHLKVASYCTTQVERSACPFCKARKLDDKFYQKLGGQFPDAVFWQELGEILRQLQKQAAEIYNQSLIELYYEIFIKGRGFANASSVEHYLSDVCYTRAAELFKNAAIASGLRGKVKSNFRLKELKNMKSGLPTTKSDNFPIPLVKQKGGQYTGFEISSHNDDFIIKIPFGRWQVKKEIDKYRPWEKFDFEQVRKSPKPISLLLSTQRRKRNKGWSKDEGTEAEIRKVMNGDYQTSYIEVKRGSKTGEKSAWMLNLSIDVPKIDKGVDPSIIGGIDVGVKSPLVCAINNALSRYSISDNDLFRFNKKMFARRRILLKKNRHKRAGHGAKNKLKPISILTGKSERFRKKLIERWACEIADFFIKNKVGTVQMENLESMKRKEDSYFNIRLRGFWPYAEMQNKIEFKLKQYGIEIRKVAPNNTSKTCSKCGHLNNYFNFEYRKKNKFPHFKCEKCNFKENADYNAALNISNPKLKSTKEEP

SEQ ID NO: 1070 - protein, 726 aa, synthetic construct
SEVEFSHEYWMRHALTLAKRARDGREVPVGAVLVLNNRVIGEGWNRAIGLHDPTAHAEIMALRQGGLVMQNYRLIDATLYVTFEPCVMCAGAMIHSRIGRVVFGVRNNKHGAAGSLVNVLNYPGMNHRVEITEGILADECAALLCDFYRMPRQVFNARKKAQSSINPGGSSGGSSGSETPGTSESATPESSGGSSGSSAKNTITKTLKLRIVRPYNSAEVEKIVADEKNNREKIALEKNKDKVKEACSKHLKVAAYCTTQVERNACLFCKARKLDDKFYQKLRGQFPDAVFWQEIGEIFRQLQKQAAEIYNQSLIELYYEIFIKGKGFANASSVEHYLSDVCYTRAAELFKNAAIASGLRGKVKSNFRLKELKNMKSGLPTTKSDNFPIPLVKQKGGQYTGFEISSHNDDFIIKIPFGRWRVKKEIDKYRPWEKFDFEQVRKSPKPISLLLSTQRRKRNKGWSKDEGTEAEIRKVMNGDYQTSYIEVKRGSKIGEKSAWMLNLSIDVPKIDKGVDPSIIGGIDVGVKSPLVCAINNALSRYSISDNDLFHFNKKMFARRRILLKKNRHRRAGHGARNKLKPITVLTEKSERFRKKLIERWACEIANFFVKNKVGTVQMENLESMKRKEDSYFNIRLRGFWPYAEMQNKIEFKLKQYGIEIRKVAPNNTSKTCSKCGHLNNYFNFEYRKKNKFPHFKCEKCNFKENADYNAALNISNPKLKSTKEEP

SEQ ID NO: 1071 - protein, 726 aa, synthetic construct
SEVEFSHEYWMRHALTLAKRARDEREVPVGAILVLNNRVIGEGWNRAIGLHDPTAHAEIMALRQGGLVMQNYRLIDATLYVTFEPCVMCAGAMIHSRIGRVVFGVRNNKHGAAGSLVNVLDYPGMNHRVEITEGILADECAALLCDFYRMPRQVFNARRKAQPSINPGGSSGGSSCCETPCASESVTPKSSGGSSAGSTKNTITKTLKLRIVRPYNSAEVEKIVADEKNSREKIALEKNKDKVKEACSEHLKVAAYCTTQVERNACLFCKARKLDDRFYQKLRGQFPDAVFWQEIGEIFRQLQKQAAEIYNQSLIELYYEIFIKGKGFANASSVEHYLSDVCYTRAAELFKNAAIASGLRGKVKSNFRLKELKNMKSGLPTTKSDNFPIPLVKQKGGQYTGFGISSHNDDFIIKIPFGRWQAKEEIDKYRPWEKFDFEQVRKSPKPISLLLSTQRRKRNKGWSKDVGTEAEIRKVMNGDYQTSYIEVKRGSKIGEKSAWMLNLSIDVPKIDKGVDPSIIGGIDVGVKSPLVCAINNAFSRYSISDNDLFRFNKKMFARRRILLKKNRHQRAGHGAKNKLKPITILTEKSGRFRKKLIERWACEIADFFIKNKVGTVQMENLESMKRREDSYFNIRLRGFWPYAEMQNKIEFKLKQYGIEIRKVTPNNTSKTCSRCGHLNNYFNFEYRKKNKFPHFKCEKCNFKENADYNAALNISNPKLKSSKEEP

SEQ ID NO: 1072 - protein, 726 aa, synthetic construct
SEVEFSHEYWMRHALTLAKRARDEREVPVGAVLVLNNRVIGEGWNRTTGLHDPTAHAEIMALRQGGLVMQNHRLVDATLYVTFEPCVMCAGAMIHSRIGRVVFGVRNSKRGAAGSLMNVLNYPGMNHCVEITEGILVDECAALLCDFYRMPCQVLNAQKKAQSSISSGGSSGGSSGSDTLGASESVTPKSSVGSSASSTKNTITKTLKLRIVRPYNSAEVEKIVADEKDNRERIALEKNKDKVKEACSKHLKVAAYCTAQVERNACLFCKARKLDDKFYQKLRDQFPDAVFWQEIGEIFRQLQKQAAEIYNQSLIELYYEIFIKGKGFANASSVEHYLSDVCYTRAAELFKNAAIASGLRGKVKSNFRLKELKNMKSGLPTTKSDNFPIPLVKQKGGQYTGFEISSHNDDFIIKIPFGRWQVKKEIDKYRPWEKFDFEQVRKSPKPISLLLSTQRRKRNKGWSKDEGTEAEIRKVMNGDYQTSYIEVKRGSKIGEKSAWMLNLSIDVPKIDKGVDPSIIGGIDVGVKSPLVCAINNAFSRYSISDNDLFRFNKKMFARRRILLKKNRHKRAGHGAKNKLKPITILTEKSVRFRKKLIERWACEIADFFIKNKVGTVQMENLESMKGKEDSYFNIRLRGFWPYAEMQNKIEFKLKQYGIEIRKVAPNNTSKTCSKCGHLNNYFNFEYRKKNKFPHFRCEKCNFKENADYNAALNISNPELKSTKEEP

SEQ ID NO: 1073 - protein, 726 aa, synthetic construct
SEVEFSHEYWMRHALTLAKRARDEREVPVGAILVLNNRVIGEGWNRAIGLHDPTAHAEIMALRQGGLVMQNYRLIDATLYVTFEPCVMCAGAMIHSRIGRVVFGVRNNKHGAAGSLVNVLNYPGMNHRVEITEGILADECAALLCDFYCMPRQVFNARKKAQSSINPGGSSGGSSGSETPGTSGSATPEGSGGSSGGSAKSTITKTLKLRIVRPYNSAEVEKIVADEKNNREKIALEKNKGKVKEACSKHLKVATYCTTQVERNACLFCKARKLDDRFYQKLRGQFPDAVFWQEIGEIFRQLQKQAAEIYNRSLIELYYEIFIKGRGFANASSVEHYLSDVCYTRAAELFKNAAIASGLRGKVKSNFRLKELKNMKSGLPTTKSDNFPIPLVKQKGGQYTGFEISSHNDDFIIKIPFGRWQVKKEIDKYRPWEKFDFEQVRKSPKPISLLLSTQRRKRNKGWSKDEGTEAEIRKVMNGDYQTSYIEVKRGSKTGEKSAWMLNLSIDVPKIDKGVDPSITGGIDVGVKSPLVCAINNALSRYSISDNDLFHFNKKMFARRRILLRKNRHKRAGHGARNKLKPVTVLTEKSERFRKKLIERWACEIANFFIKNKVGTVQMENLESMKRREDSYFNIRLRGFWPYAEMQNKIEFKLKQYGIEIRKVAPNNTSKTCSKCGHLNNYFNFEFRKKNKFPHFKCEKCNFKEDADYNAALNISNPKLKSTKEEP

SEQ ID NO: 1074 - protein, 726 aa, synthetic construct
SEVEFSHEYWMRHALTLAKRARDEREVPVGAVLVLNNRVIGEGWNRAIGLHDPTAHAEIMALRQGGLVMQNYRLIDATLYVTFEPCVMCAGAMIHSRIGRVVFGVRNSKRGAAGSLMNVLNYPGMNHCVEITEGILADECAALLCDFYCMPRQVFNAQKRAQSSINSGGSSGGSSGSETPGTSESATPESSGGGSSGSAKNTITKTLKLRIVRPYNSAEVEKIVADEKNSREKIALERNKDKVKEACSEHLKVAAYCTTQVERNACLFCKARKLDDRFYQKLRGQFPDAVFWQEIGEIFRQLQRQAAEIYNQSLIELYYEIFIKGKGIASASRVGHYLSDVCYTRAAELFKNAAIASGLRSKVRSNFRLKELKNMKSGLPTTKSDNFPIPLVKQKGGQYTGFEISSHNDDFVIKIPFGRWQVKKEIDKYRPWEKFDFEQVRKGPKPISLLLSTQRRKRNKGWSKDEGTEAEIRKVMSGDYQTSYIEVKRGSKTGEKSAWMLNLSIDVPKIDKGVDPSIIGGIDVGVRSPLVCAISNALSRYSISDNDLFHFNKKMFARRRILLKKNRHKRAGHGAKNKLKPISILTEKSERFRKKLIERWACEIADFFIKNKVGTVQMENLESMKRREDSYFNIRLRGFWPYAKMLNKIEFKLKQYGIKIRKVAPNNTSKTCSKCGHLNNYFNFEYRKKNKFPHFKCEKCNFKENADYNAALNISNPKLKSTKGES

SEQ ID NO: 1075 - protein, 726 aa, synthetic construct
SEDEFSHEYWMRHALTLAKRARDGREVPVGAVLVLNNRVIGEGWNRAIGLHDPTAHAEIMALRQGGLVMQNYRLIDATLYVTFEPCVMCAGAMVHSRIGRVVFGVRNSKRGAAGSLMNVLDYPGMGHRVEITEGILADECAALLCDFYCMPRQVFNAQKRAQSSINSGGSSGGSSGSETPGTSESATPESSGGGSSGSAKNTITKTLQLRIVRPYNSAEVEKVVADEKNNREKIALEKNKDKVKEACSKHLKVASYCTTQVERNACPFCKARKLDDKFYQKLRGQFPDAVFWQELGEILRQLQKQAAEIYNQSLIELYYEIFIKGKGFANASSVEHYLSDVCYTRAAELFKNAAIASGLRGKVKSNFRLKELKNMKSGLPTTKSDNFPIPLVKQKGGQYTGFEISSHNDDFIIKIPFGRWQVKKEIDKYRPWEKFDFEQVRKSPKPISLLLSTQRRKRNKGWGKDEGTEAEIRRVMNGDYQTSYIEVKRGSKIGEKSAWMLNLSIDVPKIDKGVDPSIIGGIDVGVKSPLVCAINNAFSRYSISDNDLFHFNKKMFARRRILLKKNRHKRAGHGAKNKLKPISILTEKSERFRKKLIEKWACEIADFFVKNKVGTVQMENLESMKRKEDSYFNIRLRGFWPYAEMQNRIEFKLKQYGIEIRKVAPNNTSKTCSKCGHLNNYFNFEYRKKNKFPHFKCEKCNFKENADYNAALNISNPKLKSTKEGP

SEQ ID NO: 1076 - protein, 726 aa, synthetic construct
SEVELSHEYWMRHALTLAKRARDEREVPVGAVLVLNNRVIGEGWNRAIGLHDPTAHAEIMALRQGGLVMQNHRLVNATLYVTFEPCVMCAGAMIHSRIGRVVFGVRNSRRGAAGSLMNVLDYPGMNHRVEITEGILADECAALLCDFYRMPRQVFNAQKKAQSSFNSGGSPGCGSGSETPGTSESAAPKSSGGSSGGSAKNTITKTLKLRIVRPYNSAEVEKIVADEKNNREKIALEKNKDKVKEACSKHLKVAAYCTTQVERNACLFCKARKLDDKFYQKLRGQFPDAVFWQEIGEVFRQLQKQAAEIYNQSLIELYYEIFIKGKGFANASSVEHYLSDVCYTRAAELFKNAAIASGLRGKVKSNFRLKELKNMKSGLPTTKSDNFPIPLVKQKGGQYTGFEISSHDDDFIIKIPFGRWQVKKEIDKYRPWEKFDFEQVRKSPKPISLLLSTQRRKRNKGWGKDEGTEAEIKKVMNGDYQTSYIEVKRGGKIGEKSAWMLNLSIDVPKIDKGVDPSIIGGIDVGVKSPLVCAINNAFSRYSISDNDLFRFNKKMFARRRILLKKSKHKRAGHGAKNKLKPITILTEKSGRFRKKLIERWACEIADFFIKNKVGTVQMENLESMKRKEDSYFNIRLRGFWPYAEMQNKIEFKLKQYGIVIRKVAPNNTSKTCSKCGHLNNYFNFEYRKKNKFPYFKCEKCNFKENADYNAALNISNPKLKSTKEEP

SEQ ID NO: 1077 - protein, 726 aa, synthetic construct
SEVEFSHEYWMRHALTLAKRARDEREVPVGAILVLNNRVIGEGWNRAIGLHDPTAHAEIMALRQGGLVMQNYRLIDATLYVTFEPCVMCAGAMIHSRIGRVVFGVRNSKRGAAGSLMNVLNYPGMNHCVEITEGILVDECAALLCDFYRMPRQVFNAQKKAQSSINSGGSSGGSSGSETPSTSESATLESSGGSSGGSAKNTITKTLKLRIVRPYNSAEVEKIVTDEKNNREKIALEKNKDKVKEACSKHLKMASYCTTQVERNACLFCKARKLDDKFYQKLRGQFPDAVFWQELGGIFRQLQKQAAEIYNQSLIELYYEIFIKGKGITNASRVEHYLSDVCYTRAAELFKNAAIASGLRSKVRSNFRLKELKNMRSGLPTTKSDNFPIPLVKQKGGQYTGFEISSHNSDFIIKIPFGRWQVKEEIDKYRPWEKFDFEQVRKSPKPISLLLSTQRRKKNRGWSKDEGTEAEIKKVMNGDYQTSYIEVKRGSKIGEKSAWMLNLSIDVPKIDKGVDPSIIGGIDVGVKSPLVCAVNNAFSRYSISDNELFHFNKKMFARRRILLKKNRHKRAGHGVKNKLKPITILTEKSGRFRKKLIERWACEIADFFVKNKVGTVQMENLESMKRKEDSYFNIRLRGFWPYAEMQNKIEFKLKQYGIKVRKVAPNNTSKTCSKCGHLNNYFSFEYRKKNKFPHFKCEKCNFKENADYNAALNISNPKLKSTKEEP

SEQ ID NO: 1078 - protein, 726 aa, synthetic construct
SEVEFSHEYWMRHALTLAKRARDEREVPVGAVLVLNNRVIGEGWNRAIGLHDPTAHAEIMALRQGGLVMQNYRLIDATLYVTFEPCVMCAGAMIHSRIGRVVFGVRNNKHGAAGSLVNVLNYPGMNHRVEITEGILADECAALLCDFYRMPRQVFNARKKARSNINSGGSSGGCSGSEMPGASESVTPKSSGGSSAGSTKNTITKTLKLRIVRPYNSAEVEKIVADEKNSREKIALERNKDKVKEACSEHLKVAAYCTTQVERNACLFCKARKLDDRFYQKLRGQFPDAVFWQETGEIFRQLQRQAAEIYNQSLIELYYEIFIKGKGFANASSVEHYLSDVCYTRAAELFKNAAIASGLRGKVKSNFRLKELKNMRSGLPTTKSDNFPIPLVKQKGGQYTGFEISSHNDDFIIKIPFGRWQVKKEIDKYRPWERFDFEQVRKSPKPISLLLSTQRRKRNKGWSKDEGTEAEIRKVMNGDYQTSYIEVKRGSKIGEKSAWMLNLSIGVPKIDKGVDPSIIGGIDVGVKSPLVCAINNAFSRYSISDNDLFHFNKKMFARRRILLKKNRHKRAGHGAKNKLKPISILTEKSKRFRKKLIERWACEIADFFIKNKVGTVQMENLESMKRKEDSYFNIRLRGFWPYAEMQNRIEFKLKQYGIEIRKVAPNNTSKSCSKCGHLNNYFNFEYRKKNKFPHFKCEKCNFKEDADYNAALNISNPKLKSTEEEP

SEQ ID NO: 1079 - protein, 726 aa, synthetic construct
SEVEFSHEYWMRHALTLAKRARDEREVPVGAILVLNNRVIGEGWNRAIGLHDPTAHAEIMALRQGGLVMQNYRLIDATLYVTFEPCVMCAGAMIHSRIGRVVFGVRNSKHGAAGSLVNVLNYPGMNHRVEITEGILADECAALLCDFYRMPRQVFGARRKAQSSINPGGSSGGSSSSETPGTSESPTPESPGGSSGGSAKNTITKTLKLRIVRPYNSAEVEKIVADEKNNREKIALEKNKDKVKEACSKHLKVAAYCTTQVERNACLFCKARKLDDKFYQKLRGQFPDAVFWQEIGEIFRQLQKQAAEIYNQSLIELYYEIFIKGRGFANASSVEHYLSDVCYTRAAELFKNAAIASGLRGKVKSNFRPKELKNMKSGLPTTKSDNFPIPLVRQKGGQYTGFEISSHNDDFIIKIPFGRWQVKKEIDKYRPWEKFDFEQVRKSPKPISLLLSTQRRKRNKGWSKDEGTEAEIRKVMNGDYQTSYIEVKRGSKTGEKSAWMLNLSIDVPKIDKGVDPSIIGGIDVGVKSPLVCAINNAFSRYSISDNDLFRFNKKMFARRRILLKKNRHKRAGHGAKNKLKPITILTGKSERFRKKLIERWACEIANFFIKNKVGTVQMENLESMKRKEDSYFNIRLRGFWPYAEMQNKIEFKLRQYGIKIRRVAPNNTSKTCSKCGHLNNYFSFEYRKKNKFPHFKCEKCNFKEDADYNAALNISNPKLKSTKEEP

SEQ ID NO: 1080 - protein, 726 aa, synthetic construct
SEVEFSHEYWMRHALTLAKRARDEREVPVGAILVLNNRVIGEGWNRAIGLHDPTAHAEIMALRQGGLVMQNYRLIDATLYVTFEPCVMCAGAMIHSRIGRVVFGVRNNKHGAAGSLVNVLNYPGMNHRVEITEGILADECAALLCDFYRMPRQVFNARKKAQSNINSGGSSGGSSGSEAPGTSESPTPESSGGSSGGSVKNTITKTLKLRIVRPYNSAEVEKIVADEKNNREKIALEKNKDKVKEACSRHLKVAAYCTTQVERNACLFCKARKLDDKFYQKLRGQFPDAVFWQEIGEIFRQLQKQAAEIYNQSLIELYYEIFIKGKGIANASSVEHYLSDVCYTRAAELFKNAAIASGLRNKIKSNFRLKELRNMKSGLPTTKSDNFPIPLVRQKGGQYTGFEISNHNGDFIIKIPFGRWQVKKEISKHRPWEKFDFEQVRKSPKPISLLLSTQRRRRNKGWGKDEGTEAEIRKVMNGDYQTSYIEVKRGSKIGEKSAWMLNLSIDVPKIDKGVDPSIVGGIDVGVKSPLVCAIDNALSRYSISDNDLFHFNKKMFARRRILLKKNRHRRAGHGVKNKLKPITILTEKSGRFRKKLIERWACEIADFFVKNKVGTVQMENLESMKRKEDSYFNIRLRGFWPYAEMQNKIEFKLKQYGIKVRKVAPNNTSKTCSKCGHLNNYFSFEYRKKNKFPHFKCEKCNFKENADYNAALNISNPKLKSTKEEP

SEQ ID NO: 1081 - protein, 726 aa, synthetic construct
SEIEFSHEYWMRRALTLAKRARDEREVPVGAVLVLNSRVIGVGWNRAISLHDPTAHAEIMALRQGGLVMQNHRLIDATLYVTFEPCVMCAGAMVHSRIGRVVFGVRNSKRGAAGSLMNVLNYPGMNHRVEITEGILADECAALLCDFYRMPRQVFNAQRKAQSSINFGGSSGGSSGSGTPGTSESATPESSGGSSGGSAKNTITKTLKLRIVRPYNSAEVEKIVADEKNKREKIALEKNKDKVKEACSKHLKVAAYCTTQVERNACLFCKARKLDDKFYRKLRGQFPDAVFWQEIGEIFRQLQKQAAEIYNQSLIELYYEIFIKGKGFANASSVEHYLSDVCYTRAAELFKNAAIASGLRGKVKSNFRLKELKNMKSGLPTTKSDNFPVPLVKQKGGQYTGFEISNHNSDFIIKIPFGRWQVKEEINKYRPWEKFDFEQVRKSPKPISLLLSTQRRKRNKGWSKDEGTEAEIRKVMNGDYQTSYIEVKRGSKIGEKSAWMLNLSIDVPKIDKGVNPSIIGGIDVGVKSPLVCAINNALSRYSISDNDLFHFNKKMFARRRILLKKNRHKRAGHGAKNKLKPITILTGKCKRFRKKLIERWACEIADFFIKNKVGTVQMENLESMKRKEDSYFNIRLRGFWPYAEMQNKIEFKLKQYGIEIRKVAPNNTSKTCSKCGHLNNYFNFEYRKRNKFPHFKCEKCNFKENADYNAALNISNPKLKSTKEEP

SEQ ID NO: 1082 - protein, 726 aa, synthetic construct
SEDEFSHEYWMRHALTLAKRARDEREVPVGAILVLNNRVIGEGWNRAIGLHDPTAHAEIMALRQGGLVMQNYRLIDATLYVTFEPCVMCAGAMIHSRVGRVVFGVRNSKHGAAGSLMNVLNYPGMNHRVEITEGILADECAALLCDFYRMPRRVFNARKKAQSSIDPGGPSGGSSGSETPGTSESATPESSGGSSGGSAKNTITKTLKLRIVRPYNSTEVEKIVADEKNNREKIALEKNKDKVKEACSKHLKVASYCTTQVERNACLFCKARKLDDKFYQKLRGQFPDAVFWQEISEIFRQLQKQAAEIYNQSLIELYYEIFIKGKGFANASRVEHYLSDVCYTRAAELFKNAAIASGLRGKVKSNFRLKELKNMKSGLPTTKSDNFPIPLVKQKGGQYTGFEISSLNDDFIIKIPFGRWQVKKEIDKYRPWEKFDFEQVRKSPKPISLLLSTQRRKRNKGWSKDEGTEAEIRKVMNGDYQTSYIEVKRGSKIGEKSAWMLNLSIDVPKIDKGVDPSIIGGIDVGVKSPLVCAINNALSRYSISDNDLFHFNKKMFARRRILLRKNRHKRAGHGAKNKLKPITMMTEKSKRFRKKLIERWACEIADFFIKNKVGTVQMENLESMKRKEDSYFNIRLRGFWPYAEMQNKIEFKLKQYGIVVRKVAPNNTSKTCSKCGHLNHYFNFEFRKKNKFPHFKCEKCNFKEDADYNAALNISNPKLKSTKEEP

SEQ ID NO: 1083 - protein, 726 aa, synthetic construct
SEVEFSHEYWMRHALTLAKRARDEREVPVGAVLVLNNRVIGEGWNRTTGLHDPTAHAEIMALRQGGLVMRNYRLTDATLYVTFEPCVMCAGAMIHSRIGRVVFGVRNSKRGAAGSLMNVLNYPGMNHCVEITEGILVDECAALLCDFYRMPRQVLNAQKKAQSSISSGGSSGGSSGSETPGASGSVIPKSSGGSSAGSTKDTITKTLKLRIVRPYNSAEVEKVVADEKNNREKIAMEKNKDKVKEACSKHLKVASYCTTQVERNACLFCKARKLDDKFYQKLRGQFPDAVFWQEIGEIFRQLQKQAAEIYNQSLIELYYEIFIKGKGFANASSVEHYLSDVCYTRAAELFKNAAIASGLRGKVKSNFRLKELKNMKSGLPTTKSDNFPIPLVRQKGGQYTGFEISSHNDDFIIKIPFGRWQVKKEIDKYRPWEKFDFEQVRKSPKPISLLLSTRRRKRNKGWSKDEGTEAEIRKVMNGDYQTSYIEVKRGSKIGEKSAWMLNLSIDVPKIDNGVDPIIVGGIDVGVKSPLVCAINNAFSRYSISDNDLFRFNKKMFARRRILLGKNRHKRAGHGVKNKLKPITILTEKSGRFRKKLIERWACEIADFFVKNKVGTVQMENLESMKRKEDSYFNIRLRGFWPYAEMQNKIEFKLRQYGIKVRKVAPNNTSKTCSKCGHLNNYFSFEYRKKNKFPHFKCEKCNFKENADYNAALNISNPKLKSTKEEL

SEQ ID NO: 1084 - protein, 726 aa, synthetic construct
SEVEFSHEYWMRRALTLAKRARDEREVPVGAVLVLNNRVIGVGWNRAVGLHDPTAHAEIMALRQGGLVLQNYRLIEATLYVTFEPCIMCAGAMIHSRIGRVVFGVRNSKRGAAGSLMNVLNYPGMNHRVEITEGILADECAALLCDYYRMPRQVFNTRKKARSKINSGGSSGGSSGSETPGASGSVTPKSSGGSSAGSTKDTITKTLKLRIVRPYNSAEVEKIVADEKNSRERIALEKNKDKVKEACSKHLKVAAYCTTLVERNACLFCKARRLDDKFYQKLRGQFPDAVFWQEVGEIFRQLQKQAAEIYNQSLIELYYEIFIKGKGFANASSVEHYLSDVCYTRAAELFKNAAIASGLRGKVKSNFRLKELKNMKSGLPTTKSDNFPIPLVKQKGGKYTGFEISSHNDDFIIKIPFGRWQVKKEIDKYRPWEKFDFEQVRKSPKPISLLLSTQRRKRNKGWGKDEGTEAEIRKVMNGDYQTSYIEVKRGSKIGEKSAWMLNLSIDVPKIDKGVDPSIIGGIDVGVKSPLVCAINNALGRYSISDNDLFHFNKKMFARRRILLRKNRHKRAGHGVRNKLKPITILTEKSKRFRKTLIERWACEIADFFIKNKVGTVQIENLESMKRKEDSYFNIRLRGFWPYAEMQNKIEFKLKQYGIEIRKVAPNNTSKTCSKCGHLNNYFNFEYRKKNKFPHFKCEKCNFKEDADYNAALNISNPKLKSTREEP

SEQ ID NO: 1085 - protein, 726 aa, synthetic construct
SEVEFSHEYWMRHALTLAKRARDEREVPVGAVLVLNNRVIGEGWNRAIGLHDPTAHAEIMALRQGGLVMQNYRLSDATLYVTFEPCVMCAGAMIHSRIGRVVFGVRNSKRGAAGSLMNVLNYPGMNHCVEITEGILMDECAALLCDFYRMPRQVLSAQEKAQSSISSGGPSGGSSCSETPGASESVTPKSSGGSSTGSTKNTITKTLKLRIVRPYNSAEVEKIVADEKNSREKIALEKNKDKVKEACSEHLKVAAYCTTQVERNACLFCKARKLDDRFYQKLRGQFPDAVFWQEIGEIFRQLQKQAAEIYNQSLIELYYEIFIKGKGFAIASSVEHYLSCVCYTRAAELFKNAAIASGLRGKVKSNFRLKELKNMKSGLPTTKSDNFPIPLVKQKGGQYTGFEISSHNDDFIIKIPFGRWQVKKEIDKYRPWEKFDFEQVRKSPKPISLLLSTRRRKRNKGWSKDEGTEAEIRKVMNGDYQTSYIEVKRGSKIGEKSAWMLNLSIDVPKIDKGVDPSIIGGIDVGVKSPLVCAINNAFSRYSISDNELFHFNKKMFARRRILLKKNRHKRAGHGAKNKLKPISILTEKSERFRKKLIEKWACEIADFFIKNKVGTVQMENLESMKRKEDSYFNIRLRGFWPYAEMQNKIEFKLKQYGIEVRKVAPNNTSKTCSKCGHLNNYFNFEYRKKNKFPHFKCEKCNFKENADYNAALNISNPKLKSTREEP

SEQ ID NO: 1086 - protein, 726 aa, synthetic construct
SEVEFSHEYWMRHALTLAKRARDEREVPVGAILVLNNRVIGEGRNRAIGLHDPTAHAEIMALRQGGLVMQNYRLIGATLYVTFEPCVMCAGAMIHSRIGRVVFGVRNNKHGAAGSLVNVLNYPGMNHRVEITEGILADECAALLCDFYRMPRQVFNARKKAQSNINPGGSSGGSSGSETPGTSESATPGGSGGSSGGSAKNTITKTLKLRIVRPYNSAEVEKIVADEKNNRERIALEKNKDKVREACSKHLKVAAYCTTLVERNACPFCKARKLDDKFYQKLRGQFPDAVFWQELGEIFRQLQKQAAEIYNQSLIELYYEIFIKGKGFANASSVEHYLSDVCYTRAAELFKNAAIASGLRGKVKSNFRLKELKNMKSGLPTTKSDNFPIPLVKQKGGQYTGFEISSHNDDFIIKIPFGRWQVKKEINKFRPWEKFDFEQVRKSPKPISLLLSTQRRKRNRGWSKDEGTEAEIKRVMNGDYQTSYIEVKRGNKIGEKSAWMLNLSIDVPKIDKGVDPSIIGGIDVGVKSPLVCAISNAFSRYSISDNDLFRFNKKMFARRRILLKKNRHKRAGHGAKNKLKPISILTEKSKRFRKKLIERWACEIADFFIKNKVGTVQMENLESMKRKEDGYFNIRLRGFWPYAEMQNKIEFKLKQYGIEIRKVAPNNTSKTCSKCGHLNNYFNFEYRKTNKFPHFKCEKCNFKEDADYNAALNISNPKLKSTKEEP

SEQ ID NO: 1087 - protein, 726 aa, synthetic construct
SEVEFSHEYWMRHALTLAKRARDEREVPVGAVLVLNNRVIGEGWNRAIGLHDPTAHAEIMALRQGGLVMQNYRLTDATLYVTFEPCVMCAGAMIHSRIGRVVFGVRNSKRGAAGSLMNVLNYPGMNHCVEITEGILVDECAALLCDFYRMPRQVLNAQKKAQSSISSGGSSGGSSGSVTPGASGSVTPKSSGGSSAGSTKDTITKTLKLRIVRPYNSAEVEKIVADEKNNREKIALEKNKDKVKEACSKHLKVASYCTTQVERNACPFCKARKLDDKFYQKLRGQFPDAVFWQELGEIFRQLQKQAAEIYNQSLIELYYEIFIKGKGFANASSVEHYLSDVCYTRAAELFKNAAIASGLRGKVKSNFRMKELKNMKSGLPTTKSDNFPIPLVKQKGGQYTGFEISNRNSDFIIKIPFGRWQVKKEINKYRPWEKFDFEQVRKSPKPISLLLSTQRRKRNKGWSKDEGTEAEIRKVMNGDYQTSYIEVKRGSRIGEKSAWMLSLSIDVPKIDRGVDPSIIGGIDVGVKSPLVCAINNALSRYSISDNDLFHFNKKMFARRRILLKKNRHRRAGHGARNKLKPITIMTEKSKRFRRKLIERWACEIADFFIKNKVGTVQMESLESMKRKEDSYFNIRLRGFWPYAEMQNKIEFKLKQYGIEIRKVAPNNTSKTCSKCGHLNNYFNFEYRKKNKFPHFKCEKCNFKENADYNAALNISNPKLKSTKEEP

SEQ ID NO: 1088 - protein, 726 aa, synthetic construct
SEVEFSHEYWMRHALTLAKRARDEREVPVGAILVLNNRVIGEGWNRAIGLHDPTAHAEIMALRQGGLVMQNYRLIDATLYVTFEPCVMCAGAMIHSRIGRVVFGVRNSKHGAAGSLVNVLNYPGMNHRVEITEGILADECAALLCDFYRMPRQVFNARKKAQSSINPSGSSGGSSGSATPGTSESATPESSGGGFGSSAKNTITKTLQLRIVRPYNSAEVEKIVADEKNNREKIALEKNKDKVKEACSKHLKVASYCTTQVERNACLFCKARKLDDKFYQKLRGQFPDAVFWQEIGEIFRQLQKQAAEIYNQSLIELYYEIFIKGKGFANASSVEHYLSDVCYTRAAELFKNAAIASGLRGKVKSNFRLKELKNMKSGLPTTKSDNFPIPLVKQKGGQYTGFEISSHNDDFIIKIPFGRWQVKKEINKYRPWEKFDFEQVRRSPKPISLLLSTQRRKRNKGWSKDEGTEAEIRKVMNGDYQTSYIEVKRGSKTGEKSAWMLNLSIDVPKIDKGVDPSIIGGIDVGVKSPLVCAVNNAFSRYSISDNDLFHFNKKMFARRRILLKKNRRRRAGHGAKNKLKPITILTEKSVRFRKKLIERWACEIADFFIKNKVGTVQMENLESMKRKEDSYFNIRLRGFWPYAEMQNKIEFKLKQYGIKIRKVAPNNTSKTCSKCGHLNNYFSFEYRKKNKFPHFKCEKCNFKEDADYNAALNISNPKLKSTKEEP

SEQ ID NO: 1089 - protein, 726 aa, synthetic construct
SEVEFSHEYWMRRALTLAKRARDEREVPVGAVLVLNNRVIGVGWNRAVGLHDPTAHAEIMALRQGGLVMQNYRLIEATLYVTFEPCIMCAGAMIHSRIGRVVFGVRNSKRGAAGSLMNVLDYPGMGHRVEITEGILADECAALLCDFYCMPRQVFNAQKRAQSSINSGGSSGGSSGSDTPGTSESATLESSGGSSGGSAKNTITKTLKLRIVRPYNSAEVERIVADEKNSREKIALEKNKDKVREACSKHLKVASYCTTQVERNACPFCKARKLDDKFYQKLRGQFPDAVFWQEIGEIFRQLQKQAAEIYNQSLIELYYEIFIKGRGFANASSVEHYLSDVCYTRAAELFKNAAIASGLRGKVKSNFRLKELKNMKSGLPTTKSDNFPIPLVKQKGGQYTGFEISSHNDDFIIKIPFGRWQVKKEVDKYRPWEKFDFEQVRKSPKPISLLLSTQRRKRNKGWSKDEGTEAEIRKVMNGDYQTSYIEVKRGSKIGEKGAWMLSLSIDVPKIDKGVDPRIIGGIDVGVKSPLVCAINNAFSRYSISDNDLFHFNKKMFARRRILLKKNRHKRAGHGAKNKLKPITILTEKSVRFRKKLIERWACEIADFFIKNKVGTVQMENLESMKRKEDSYFNIRLRGFWPYAEMQNKIEFKLKQYGIEIRKVAPNNTSKTCSKCGHLNNYFNFEYRRRNKFPHFKCEKCNFKEDADYNAALNISNPKLKSTKEEP

SEQ ID NO: 1090 - protein, 726 aa, synthetic construct
SEVEFSHEYWMRHALTLAKRARDEREVPVGAVLVLNNRAIGEGWNRAIGLHDPTAHAEIMALRQGGLVMQNYRLTDATLYVTFEPCVMCAGAMIHSRIGRVVFGVHNSKRGAAGSLMNVLNYPGMNHCVEITEGILVDECAALLCDFYRMPRQVLNAQKKAQSSISSGGLSGGSSGSETPGASGSVTPKSSVGSSAGSTKNTITKTLKLRIVRPYNSAEVEKIVADEKNNREKVALEKNKDKVKEACSKHLKVASYCTTQVERNACPFCKARKLDDKFYQKLRGQFPDAVFWQELGEIFRQLQKQAAEIYNQSLVELYYEILIKGKGIANASSVEHYLSDVCYTRAAELFKNAAIASGLRNKIKSNFRLKELRNMKSGLPTTKSDNFPIPLVRQKGGQYTGFEISNHNGDFIIKIPFGRWQVKKEINKHRPWEKFDFEQVRKSPKPISLLLSTQRRKRNKGWSKDEGTEAEIRKVMNGDYQTSYIEVKRGSKIGEKSAWMLNLSIDVPKIDKGVDPSIIGGIDVGVKSPLVCAINNAFSRYSISDNDLFRFNKKVFARRRILLKKNRHKRAGHGTKNKLKPITILTEKSGRFRKKLIERWACEVANFFIKNKVGTVQMENLESMKRKEDSYFNIRLRGFWPYAEMQNKIEFKLKQYGIKIRKVAPNNTSKTCSKCGHLNNYFSFEYRKRNKFPHFKCEKCNFKEDADYNAALNISNPKLKSTKEGL

SEQ ID NO: 1091 - protein, 726 aa, synthetic construct
SEVEFSHEYWMRHALSLAKRARDEREVPVGAVLVLNNRIIGEGWNRAIGLHDPTAHAEIMALRQGGLVMQNYRLADATLYVTFEPCVMCAGAMVHSRIGRVVFGVRNSKRGAAGSLMNVLNYPGVNHRVEITEGILVDECAALLCDFYRMPRQVLNAQKKAQSSISSGGSSGGCSGSEMPGASESVTPKSSGGSSAGSTKNTITKTLKLRIVRPYNSAEVEKIVADEKNSREKIALERNKDKVKEACSKHLKVAAYCTTQVERNACLFCKARKLDDKFYQKLRGQFPDAVFWQEIGEIFRQLQKQAAEVYNQSLIELYYEIFIKGKGFANASNVEHYLSDVCYTRAAELFKNAAIASGLRGKVKSNFRLKELKNMKSGLPTTKSDNFPIPLVKQKGGQYTGFEISSHNDDFIIKIPFGRWQVKKEIDKYRPWEKFDFEQVRKSPKPISLLLSTQRRKRNKGWSKDEGTEAEIRKVMNGDYQTSYIEVKRGSKIGEKSAWMLNLSIDVPKIDKGVDPSIIGGIDVGVKSPLVCAINNAFSRYSISDNDLFHFNKKMFARRRILLKKNRHKRAGHGAKNKLKPISILTEKSKRFRKKLIERWACEIADFFVKNKVGTVQMENLESMKRKEDSYFNIRLRGFWPYAEMQNKIEFKLKQYGIKVRKVAPNNTSKTCSKCGHLNNYFSFEYRKMNKFPHFKCEKCNFKENADYNAALNISNPKLKSAKEEP

SEQ ID NO: 1092 - protein, 726 aa, synthetic construct
SEVEFSHEYWMRHALTLAKRARDEREVPVGAVLVLNNRVIGVGWNRAVGQHDPTAHAEIMALRQGGLVMQNYRLIEATLYVTFEPCIMCAGAMIHSRIGRVVFGVRNSKRGAAGSLMNVLNYPGMNHRVEITEGILADECAALLCDYYRMPRQVFNARKKAQSSINSGGSSDGGSGSVTPGTSESATPKSSGGSSAGSTKNTITKTLKLRIVRPYNSAEVEKIVSDEKNNRERIALERNKDKVKEACSEHLKVAAYCTTQVERNACLFCKARKLDDKFYQKLRGQFPDAVFWQEIGEIFRQLQKQAAEIYNQSLIELYYEIFIKGKGFANASSVEHYLSDVCYTRAAELFKNAAIASGLRGKVRSNFRLKELKNMKSGLPTTKSDNFPIPLVKQKGGQYTGFEISSHNDDFIIKIPFGRWQMKKEIDRYRPWEKFDFEQVRKSPKPISLLLSTQRRKRNKGWSKDEGTEAEIRKVMNGDYQTSYIEVKRGSKIGEKSAWMLNLSIDVPKIDKGVDPSIIGGIDVGVKSPLVCAINNAFSRYSISDNDLFHFNKKMFARRRILLKKNRRRRAGHGAKNKLKPITILTEKSVRFRKKLIERWACEIADFFIKNKVGTVQMENLESMKRKEDSYFNIRLRGFWPYAEMQNKIEFKLKQYGIEIRRVAPNNTSRTCSKCGHLNNYFNFEYRRKYKFPHFKCEKCNFKEDADYNAALNISNPKLKSTKEEP

SEQ ID NO: 1093 - protein, 726 aa, synthetic construct
SEVEFSHEYWMRRALTLAKRARDEREVPVGAVLVLNNRVIGVGWNRAVGLHDPTAHAEIMALRQGGLVMQNYRLIEATLYVTFEPCIMCAGAMIHSRIGRVVFGVRNSKHGAAGSLMNVLNYPGMNHRVEITEGILADECAALLCDFYRMPRRVFNARKKAQSSISPGGSSGGSSGSETPGASENVTPRSSGGSSGGSAKNTITKTLKLRIVRPYNSAEVEKTVADEKNNRERIALEKNKDKVKEACSKHLKVAAYCTTQVERNACLFCKARKLDDKFYQKLRGQFPDAVFWQEIGEIFRQLQRQAAEIYNQSLIELYYEIFIKGKGFANASSVEHYLSDVCYTRAAELFKNAAIASGLRGKVKSNFRLKELKNMKSGLPTTKSDNFPIPLVKQKGGQYTGFEISSHNDDFIIKIPFGRWQAKKEIDKYRPWEKFDFEQVRKSPKPISLLLSTRRRKRNKGWSKDEGTEAEIRRVMNGDYQTSYIEVKRGSKIGEKSAWMLNLSIDVPKIDKGVDPSIIGGIDVGVKSPLVCAINNAFSRYSISDNDLFHFNKKMFARRRILLKKNRHKRAGHGTKNKLKPISILTEKSKRFRKKLIERWACEIADFFIKNKVGTVQMENLESMKRKEDSYFNIRLRGFWPYAEMQNKIEFKLKQYGIEIRKVAPSNTSKTCSKCGHLNNYFNFEYRRKNKFPHFKCEKCNFKENADYNAALNISNPKLKSTKEEP

SEQ ID NO: 1094 - protein, 726 aa, synthetic construct
SEVEFSHEYWMRHALTLAKRARDEREVPVGAILVLNNRVIGEGWNRAIGLHDPTAHAEIMALRQGGLVMQNYRLIDATLYVTFEPCVMCAGAMIHSRIGRVVFGVRNNKHGAAGSLVNVLNYPGMNHRVEITEGILADECAALLCDFYRMPRQVFNARKKAQSSINPGGSSGGSSGSETPGTSESATPESSGGSSGSSAKNTITKTLKLRIVRPYNSAEVEKIVADEKNNREKIALEKNKDKVKEACSKHLKVAAYCTTQVERNACLFCKARRLDDKFYQKLRGQFPDAVFWQEIGEIFRQLQKQAAEVYNQSLVELYYEILIKGKGIANASSVEHYLSNVCYTRAAELFKNAAIASGLRNKIKSNFRLKELRNMKSGLPTTKSDNFPIPLVRQKGGQYTGFEISNHDGDFIIKIPFGRWQVKKEINKYRPWEKFDFEQVRKSPKPISLLLSTQRRKRNKGWSKDEGTEAEIRKVMNGDYQTSYIEVKRGSKIGEKSAWMLNLSIDVPKIDKGVDPSIIGGIDVGVKSPLVCAINNALSRYSISDNDLFHFNKKMFARRRILLRKNRHKRAGHGAKNKLKPITTMTEKSRRFRKKLIERWACEIADFFIKNKVGTVQMENLESMKRKEDSYFNIRLRGFWPYAEMQNKIEFKLKQYGIVVRKVAPNNTSKTCSKCGHLNNYFNFEYRKKNKFPHFKCEKCNFKENADYNAALNISNPKLKSTKGEP

SEQ ID NO: 1095 - protein, 726 aa, synthetic construct
SEVEFSHEYWMRHALTLAKRARDEREVPVGAVLVLNNRVIGEGWNRAIGLHDPTAHAEIMALRQGGLVMQNYRLVDATLYVTFEPCVLCAGAMVHSRIGRVVFGVRNSKRGAAGSLMNVLNYPGMNHRVEITEGILADECAALLCDFYRMPRQVFNARKKAQSSINPSGSSGGSSGSVTPGTSESATPESSGGGFGGSAKNTITKTLKLRIVRPYNSAEVEKIVADEKNNREKIALEKNKDKVKEACSKHLKVAAYCTTQVERNACLFCKARRLDDKFYQKLRGQFPDAVFWQEIGEIFRQLQKQAAEVYNQSLVELYYEILIKGKGFANASSVEHYLSDVCYTRAAELFKNAAIASGLRGKVKSNFRLKELKNMKSGLPTTKSDNFPIPLVKQKGGQYTGFEISSHNDDFIIKIPFGRWQAKKEIDKYRPWEKFDFEQVRKSPKPISLLLSTQRRKRNKGWSKDEGTEAEIRKVMNGDYQTSYIEVKRGSKIGEKSAWMLNLSIDVPKIDKGVDPSIVGGIDVGVKSPLVCAINNALSRYSISDNDLFHFNKKMFARRRILLRKNRHKRAGHGARNKLKPITVLTEKSERFRKKLIERWACEIANFFIKNKVGTVQMENLESMKRREDSYFNIRLRGFWPYAEMQNKIEFKLKQYGIKIRKVAPNNTSKTCSKCGHLNNYFNFEFRKKNKFPHFKCEKCNFKENADYNAALNISNPKLKSTKEEP

SEQ ID NO: 1096 - protein, 726 aa, synthetic construct
SEDEFSHEYWMRHALTLAKRARDEREVPVGAVLVLNNRVIGEGWNRAIGLHDPTAHAEIMALRQGGLVMQNHRLVDATLYVTFEPCVLCAGAMVHSRIGRVVFGVRNSKRGAAGSLMNVLNYPGMNHRVEITEGILADECAALLCDFYRMPRQVFNARKKARSNINSGGSSGGSSGSETPGASESVTPKSSGGSSGGSAKNTITKTLKLRIVRPYNSAEVEKIVADEKNNREKIALEKNKGKVKEACSKHLEVAAYCTTQVERNACLFCKARKLDDKFYQKLRGQFPDAVFWQELGEIFRQLQKQAAEIYNQSLIELYYEIFIKGKGITNASSVEHYLSDVCYTRAAELFKNAAIASGLRNKVKSNFRLKELRSMKSGLPTTKSDNFPIPLVRQKGGQYTGFEISNHNSDFIIKIPFGRWQAKKEIDKYRPWEKFDFEQVRKSPKPISLLLSTQRRKRNRGWSKDESTEAEIKKVMNGDYQTSYIEVKRGSKTGEKSAWMLNLSIDVPKIDKGVDPSIIGGIDVGVKSPLVCAINNALSRYSISDNDLFHFNKKMFARRRILLKKNRHKRAGHGAKNKLKPISILTEKSERFRKKLIERWACEIADFFIKNKVGTVQMENLESMKRREDSYFNIRLRGFWPYAKMLNKIEFKLKQYGIEIRKVAPNNTSKTCSKCGHLNNYFNFEYRKKNKFPHFKCEKCNFKENADYNAALNISNPKLKSTKGEP

SEQ ID NO: 1097 - protein, 726 aa, synthetic construct
SEVEFSHEYWMRHALTLAKRARDEREVPVGAILVLNNRVIGEGWNRAIGLHDPTAHAEIMALRQGGLVMQNYRLIDATLYVTFEPCVMCAGAMIHSRIGRVVFGVRNNKHGAAGSLVNVLNYPGMNHRVEITEGILADECAALLCDFYRMPRQVFNARKKAQSSINPGGSSGGSSGSETPGTSESATPESSGGSSGGSAKNTITKTLKLRIVRPYNSAEVEKIVADEKDSREKIALEKNRDKVKEACSKHLKVAAYCTTQVERNACLFCKARKLDDKFYQKLRGQFPDAVFWQEIGEIFRQLQKQAAEIYNQSLIELYYEIFIKGKGFANASSVEHYLSDVCYTRAAELFKNAAIASGLRGKVKSNFRLKELKNMKSGLPTTKSDNFPIPLVKQKGGQYTGFEISSHNDDFLIKIPFGRWQVKEEIDKYRPWEKFDFEQVRKSPKPISLLLSTQRRKRNKGWSKDEGTEAEIRKVMNGDYQTSYIEVKRGGKIGEKSAWMLSLSIDVPKIDKGVDPSIIGGIDVGVKSPLVCAINNAFCRYSISDNDLFHFNKKMFARRRILLKKSRHKRAGHGAKNKLKPISILTEKSKRFRKKLIERWACEIADFFIKNKVGTVQMENLESMKRKEDSYFNIRLRGFWPYAEMQNKIEFKLKQYGIEIRKVAPNNTSKTCSKCGHLNNYFNFEYRKKNKFPHFKCEKCNFKENADYNAALNISNPKLKSTKEKP

SEQ ID NO: 1098 - protein, 726 aa, synthetic construct
SEVEFSHEYWMRHALTLAKRARDEREVPVGAILVLNNRVIGEGWNRAIGLHDPTAHAEIMALRQGGLVMQNYRLIDATLYVTFEPCVMCAGAMIHSRIGRVVFGVRNSKHGAAGSLMDVLNYPGMNHRVEITEGILADECAALLCDFYRMPRQVFSARKKAQSSINPGGSSGGSSGSKTPGTSESATPESSGGSSGGSAKNSITKTLKLRIVRPYNSAEVEKIVADEKNNREKIALEKNKGKVKEACSKHLKVATYCTTQVERNACLFCKARKLDDKFYQELRGQFPDAVFWQELGEIFRQLQKQAAEIYNQSLIELYYEIFIKGKGFANASSVEHYLSDVCYTRAAELFKNAAIASGLRGKVKSNFRLKELKNMKSGLPTTKSDNFPIPLVKQKGGQYTGFEISSHNDDFIIKIPFGRWQVKKEIDKYRPWEKFDFEQVRKSPKPISLLLSTQRRKRNKGWSRDEGTEAEIRKVMNGDYQTSYIEVKRGSKIGEKSAWMLNLSIDVPKIDKGVDPSIIGGIDVGVKSPLVCAINNASSRYSISDNDLFHFNKKVFARRRILLKKNRHKRAGHGAKNKLKPITILTEKSKRFRKKLIERWACEIADFFVKNKVGTVQMENLESMKRKEDSYFNIRLRGFWPYAEMQNKIEFKLKQYGIEIRKVAPNNTSKTCSKCGHLNNYFNFEYRKKNKFPHFKCEKCNFKENADYNAALNICNPKLKSTKEEP

SEQ ID NO: 1099 - protein, 726 aa, synthetic construct
SEAEFSHEYWMRHALTLAKRARDEREVPVGAVLVLNNRVIGEGWNRAIGLHDPTAHAEIMALRQGGLVMQNYRLTDATLYVTFEPCVMCAGAMIHSRIGRVVFGVRNNKHGAAGSLVNVLNHPGMNHRVETTEGILADECAALLCDFYRMPRQVFNARKKAQSNTNSGGSSGGSSGSETPGTSESATPESSGGGSGGSAKNTITKTLKLRIVRPYNSAEVEKIVADEKNNREKIALEKNKDKVKEACSKHLKVASYCTTQVERNACLFCKARKLDDKFYQKLRGQFPDAVFWQELGEIFRQLQKQAAEIYNQSLIELYYEIFIESKGFANASSVEHYLSDVCYTRAAELFKNAAIASGLRGKVKSNFRLKELKNMKSGLPTTKSDNFPIPLVKQKGGQYTGFEISSHNDDFIIKIPFGRWQVKKEIDRYRPWEKFDFEQVRKSPKPISLLLSTQRRKRNKGWSKDEGTEAEIRKVMNGDYQTSYIEVKRGSKIGEKSAWILNLSIDVPKIDKGVDPSIIGGIDVGVKSPLVCAINNAFSRYSISDNDLFRFNKKVFARRRILLKKNRYKRAGHGTKNKLKPITILTEKSGRFRKKLIERWACEIANFFIKNRVGTVQMENLESMKRKEDSYFNIRLRGFWPYAEMQNKIEFKLKQYGIEIRKVAPNNTSKTCSKCGHLNNYFSFEYRKKNKFPHFKCEKCNFKEDADYNAALNISNPKLKSTKEEP

SEQ ID NO: 1100 - protein, 726 aa, synthetic construct
SEVEFSHEYWMRHALTLAKRARDEREVPVGAILVLNNRVIGEGWNRAIGLHDPTAHAEIMALRQGGLVMQNYRLTEATLYVTFEPCVMCAGAMIHSRIGRVVFGVRNSKRGAAGSLMNVLNYPGMNHCVEITEGILVDECAALLCDFYRMPRQVLNAQKKAQSSISSGGSSGGSSGSETPGASESATPKSSVGSSAGSTKNTITKTLKLRIVRPYNSAEVEKIVADEKNNREKIALEKNKDKVKEACSKHLKVAAYCTTQVERNACLFCKARKLDDKFYQKLRGQFPDAVFWQELGEIFRQLQKQAAEIYNQSLIELYYEIFIKGKGFANASSVEHYLSDVCYTRAAELFKNAAIASGLRGKVKSNFRLKELKNMKSGLPTTKSDNFPIPLVKQKGGQYTGFEISSHNDDFIIKIPFGRWQVKKEIDKYRPWEKFDFGQVRKSPKPISLLLSTQRRKRNKGWSKDEGTEAEIRKVMNGDYQTSYIEVKRGSRIGEKSAWMLNLSIDVPKIDKGVDPSIIGGIDVGVKSPLVCAINNAFSRYSISDNDLFHFNKKMFARRRILLKKNRHKRAGHGAKNKLKPISILTEKSKRFRKKLIERWACEIADFFIKNKVGTVQMENLESMKRKEDSYFNIRLRGFWPYAEMQSKIEFKLKQYGIEIRRVAPNNTSKTCSKCGHLNNYFNFEYRKMNKFPHFKCEKCNFKENADYNAALNISNPKLKSTKEEP

SEQ ID NO: 1101 - protein, 726 aa, synthetic construct
SEVEFSHEYWMRHALTLAKRARDEREVPVGAILVLNNRVIGEGWNRAIGLHDPTAHAEIMALRQGGLVTQNYRLIDATLYVTFEPCVMCAGAMIHSRIGRVVFGVRNSKHGAAGSLVNVLNYPGMNHRVEITEGVLADECAALLCDFYRMPRQVFNARKKAQSNINPGGSSGGSSGSETPGTSDSATPGSSGGSSGGSAKNTITKTLKLRIVRPYNSAEVEKIVADEKNNREKTALEKNKDKVKEACSEHLKVATYCTTQVERNACLFCKARKLDDKFYQKLRGQFPDAVFWQEIGEIFRQLQKQAAEIYNQSLIELYYEIFIKGKGFANASSVEHYLSDVCYTRAAELFKNAAIASGLRNKTKSNFRLKELRSMKSGLPTTKSDNFPIPLVKQKGGQYTGFEISNHNSDFIIKIPFGRWQAKKEIDKYRPWEKFDFEQVRKSPKPISLLLSTQRRKRNKGWSKDEGTEAEIEKVMNGDYQTSYIEVKRGSKTGGKSAWMLNLSIDVPKIDKGVDPCIIGGIDVGVKSPLVCAINDAFSRYSISDNDLFHFNKKMFARRRILLKKNGHKRAGHGAKNKLKPITIMTEKSKRFRKKLIERWACEIADFFIKNKVGTVQMENLESMKRKEDSYFNIRLRGFWPYAEMQNKIEFKLKQYGIVVRKVAPNNTSKTCSKCGHLNNYFNFEYRKKNKFPHFKCEKCNFKENADYNAALNISNPQLKSTKGEP

SEQ ID NO: 1102 - protein, 726 aa, synthetic construct
SEDEFSHEYWMRHALTLAKRARDGREVPVGAVLVLNNRVIGEGWNRAIGLHDPTAHAEIMALRQGGLVMQNYRLIDATLYVTFEPCVMCAGAMVHSRIGRVVFGVRNSKRGAAGSLMNVLDHPGMGHRVEITEGILADECAALLCDFYRMPRQVFNAQKKARPYINSGGSSGGSSGSETPGTSESPTPESSGGSSGGSAKNTITKTLKLRIVRPYNSAEVEKIVADEKNNREKIALERNKDKVKEACSKHLKVAAYCTTQVERNACLFCKARKLDDKFYQKLRGQFPDAVFWQEIGEIFRQLQKQAAEIYNQSLIELYYEIFIKGKGFANASSVEHYLSDVCYTRAAGLFKNAAIASGLRGKVKSNFRLKELKSMKSGLPTTKSDNFPIPLVKQKGGQYTGFEISSHNDDFIIKIPFGRWQVKEEIDKYRPWEKFDFEQVRKNPKPISLLLSTQRRKRNKGWSKDEGTEAEIRKVMNGDYQTSYIEVKRGSKIGEKSAWMLNLSIDVPKIDKGVDPSIIGGIDVGVKSPLVCAINNAFSRYSISDNDLFRFNKKMFARRRILLKKNRHKRAGHGAKNKLKPISILTGKSERFRKKLIERWACEIADFFIKNKVGTVQMENLESMKRKEDSYFNIRLRGFWPYAEMQNKIEFKLKQYGIEIRKVAPNNTSRTCSKCGHLNNYFNFEYRKKNKFPHFKCEKCNFKEDADYNAALNISNPKLKSTKEEH

SEQ ID NO: 1103 - protein, 726 aa, synthetic construct
SEVEFSHEYWMRHALTLARRARDEREVPVGAVLVLNNRVIGEGWNRAIGLHDPTAHAEIMALRQGGLVMQNHRLTDATLYVTFEPCVMCAGAMIHSRIGRVVFGVRNSKRGAAGSLMNVLNYPGMNHCVEITEGILVDECAALLCDFYRMPRQVLNAQKKAQSSISSGGPSGGSSGSETPGASESATPKSSGGSSAGSTKNTIAKTLKLRIVRPYNSAEVEKIVADEKNNREKIALEKNKDKVKEACSKHLKVAAYCTTQVERNACLFCKARKLDDKFYQKLRGRFPDAVFWQELGEIFRQLQRQAAEIYNQSLIELYYEIFIKGKGFANASSVEHYLSDVCYTRAAELFKNAAIASGLRGKVKSNFRLKELRSMKSGLPTTKSDNFPIPLVKQKGGQYTGFEISNHNSDFIIKIPFGRWQVKKEIDKYRPWEKFDFEQVRKSPKPISLLLSTQRRKRNKGWSKDEGTEAEIRKVMNGDYQTSYIEVKRGSKTGEKSAWMLNLSIDVPKIDKGVDPSIIGGIDVGVKSPLVCAINNALSRYSISDNDLFRFNKKMFARRRILLKKNRHKRAGHGAKNKLKPISILTGKSERFRKKLIERWACEIADFFVKNKVGTVQMENLESMKRKEDSYFNIRLRGFWPYAEMQNKIEFKLKQYGIKVRKVAPNNTSKTCSKCGHLNNYFSFEYRKKNKFPHFKCEKCNFKENADYNAALNISNPKLKSTKEEP

SEQ ID NO: 1104 - protein, 726 aa, synthetic construct
SEVEFSHEYWMRHALTLAKRARDEREVPVGAVLVLNNRVIGEGWNRAIGLHDPTAHAEIMALRQGGLVMQNYRLIDATLYVTFEPCVMCAGAMVHSRIGRVVFGVRNSKRGAAGSLMNVLNYPGMNHRVEITEGILVDECAALLCDFYRMPCQVLNAQKKAQSSINSGGSSGGGSGGETPGTSESATQESSGGSSGGSAKNTITKTLKLRIVRPYNSAEVEKIVADEKNNREKIALEKNKDKVKEACSKHLKVAAYCTTQVERNACLFCKARKLDDKFYQKLRGQFPDAVFWQELGEILRQLQKQAAEIYNQSLIELYYEIFIKGRGFANASSVEHYLSDVCYTRAAELFKNAAIASGLRGKVKSNFRLKELKNMKSGLPTTKSDNFPIPLVKQKGGQYTGFEISSHNDDFIIKIPFGRWQVKKEIDKYRPWEKFDFEQVRKSPKPISLLLSTQRRKRNKGWSKDEGTEAEIRKVMNGDYQTSYVEVKRGSKTGEKSAWMLNLSIDVPKIDKGVDPSIIGGIDVGVKSPLVCAINNAFSRYSISDNDLFRFNKKVFARRRILLKRNRHKRAGHGAKNKLKPISILTGKSERFRKKLIERWACEIADFFIKNKVGTVQMENLESMKRREDSYFNIRLRGFWPYAEMQNKIEFKLKQYGIEIRKVAPNNTSKTCSKCGHLNNYFNFEHRKKNKFPHFKCEKCNFKENADYNAALNISNPKLKSTKEEP

SEQ ID NO: 1105 - protein, 726 aa, synthetic construct
SEVEFSHEYWMRHALTLAKRARDEREVPVGAVLVLNNRVIGEGWNRTTGLHDPTAHAEIMALRQGGLVMQNHRLVDATLYVTFEPCVMCAGAMIHSRIGRVVFGVRNSKRGAAGSLTNVLNYPGMNHRVEITEGILVDECAALLCDYYRMPRQVFNARKKAQSSINSGGSSGGSSGSETPGTSESATPESSGGSSGGSAKNTITKTLTLRIVRPYNSAEVEKIVADEKNNREKIALEKNKDKVKEACSEHLKVATYCTTQVERNACPFCKARKLNDKFYQKLRGQFPDAVFWQELGEIFRQLQKQAAEIYNQSLIELYYEIFIKGKGFANASSVEHYLSDVCYTRAAELFKNAAIASGLRGKVKSNFRLKELKNMKSGLPTTKSDNFPIPLVKQKGGQYTGFEISNHNSDFIIKIPFGRWQVKKEVDKYRPWEKFDFEQVRKSPKPISLLLSTQRRKRNKGWSKDEGTEAEIKKVMNGDYQISYIEVKRGSKIGEKSAWMLSLSVDVPKIDKGVDPSIIGGIDVGVKSPLVCAINNALSRYSISDNDLFHFNKKMFARRRILLRKNRHKRAGHGAKSKLKPITILTEKGERFRKKLIERWACEIANFFIKNKVGTVQMENLESMKRKEDSYFNIRLRGFWPYAEMQNKIEFKLKQYGIEIRKVAPNNTSKTCSRCGHLNNYFNFEYRRKNKFPHFKCEECNFKENADYNAALNISNPKLKSTKEEP

SEQ ID NO: 1106 - protein, 726 aa, synthetic construct
SEVEFSHEYWMRHALTLAKRARDEREVPVGAILVLNNRVIGEGWNRAIGLHDPTAHAEIMALRQGGLVMQNYRLIDATLYVTFEPCVMCAGAMIHSRIGRVVFGVRNNKHGAAGSLVNVLNYPGMNHRVEITEGILADECAALLCDFYRMPRQVFNARKKAQSSINPGGSSGGSSGSETPGTSESATPESSGGSSGGSAKNTITKTLKLRIVRPYNSAEVEKIVADEKNNREKIALEKNKDKVKEACSKHLKVASYCTTQVERNACPFCKARKLDDKFYQKLRGQFPDAVFWQELGEILRQLQKQAAEIYNQSLIELYYEIFIKGRGFANAGSVEHYLSDVCYTRAAELFKNAAIASGLRGKVKSNFRLKELKNMKSGLPTTKSDNFPIPLVKQKGGQYTGFEISSHNDDFVIKIPFGRWQVKKEIDKYRPWEKFDFEQVRKSPKPISLLLSTQRRKRNRGWSKDEGTEAEIRKVMNGDYQTSYIEVKRGSKIGEKSAWMLNLSIDVPKIDKGVDPSIIGGIDVGVKSPLVCAISNAFSRYSISDNDLFHFNKKMFARRRILLKKSKHKRAGHGAKNKLKPITILTEKSRRFRRKLIERWACEIADFFIKNKVGTVQMENLESMKRKEDSYFNVRLRGFWPYAEMQNKIEFKLKQYGIEIRKVAPNNTSKTCSKCGHLNNYFNFEYRRKNKFPHFKCEKCNFKENADYNAALNISNPKLKSTKEEP

SEQ ID NO: 1107 - protein, 726 aa, synthetic construct
SEVEFSHEYWMRHALTLAKRARDEREVPVGAVLVLNNRVIGEGWNRAIGLHDPTAHAEIMALRQGGLAMQNYRLVDATLYVTFEPCVLCAGAMVHSRIGRVVFGVRNSKRGAAGSLMNVLNYPGMNHRVEITEGILADECAALLCDFYRMPRQVFNARKKAQSSINPGGSSGGSSGSETPGTSESATPESSGGSPGGSAKNTITKTLKLRIVRPYNSAEVEKIVADEKDNREKIALEKNKDKVKEACSKHLKVAAYCTTQVERNACLFCKARKLDDKFYQKLRGQFPDAVFWQEIGEIFRQLQRQAAEIYNQSLIELYYEIFIKGKGFANASSVEHYLSDVCYTRAAELFKNAAIASGLRGKVKSNFRLKELKNMKSGLPTTKSDNFPIPLVKQKGGQYTGFEISSHNDDFIIKVPFGRWQAKKEIDKYRPWEKFDFEQVRKSPKPISLLLSTQRRKRNKGWSKDEGTEAEIRKVMNGDYQTSYIEVKRGSKIGEKSAWMLSLSIDVPKIDKGVDPSIIGGIDVGVKSPLVCAINNAFCRYSISDNDLFHFNKKMFARRRILQKKSRHKRAGHGAKNKLKPISILTEKSKRFRKKLIERWACEIADFFIKNKVGTVQMENLESMKRKEDSYFNIRLRGFWPYAEMQNKIEFKLKQYGIEIRKVAPNNTSKTCSKCGHLNNYFNFEYRKKNKFPHFKCEKCNFKENADYNAALNISNPKLKSTKEEP

SEQ ID NO: 1108 - protein, 726 aa, synthetic construct
SEVEFSHEYWMRHALTLAKRARDEREVPVGAILVLNNRVIGEGWNRAIGLHDPTAHAEIMALRQGGLVMQNYRLIDATLYVTFEPCVMCAGAMIHSRIGRVVFGVRNNKHGAAGSLVNVLNYPGMNHRVEITEGILADECAALLCDFYRMPRQVFNARKKAQSSINPGGSSGGSSGSETPGTSESATPESSGGSSGSSAKNTITKTLKLRIVRPYNSAEVEKIVADEKNNREKIALEKNKDKVKEACSKHLKVAAYCTTQVERNACLFCKARRLDDKFYQKLRGQFPDAVFWQEIGEIFRQLQKQAAEVYNQSLVELYYEILIKGKGIANASSVEHYLSDVCYTRAAELFKNAAIASGLRNKIKSNFRLKELRNMRSGLPTTKSDNFPIPLVRQKGGQYTGFEISNHDGDFIIKIPFGRWQVKKEINKHRPWEKFDFEQVRKSPKPISLLLSTQRRKRNKGWSKDEGTEAEIRKVMNGDYQTSYIEVKRGSKIGEKSAWMLNLSIDVPKIDKGVDPSIIGGIDVGVKSPLVCAINNALSRYSISDNDLFHFNKKMFARRRILLRKNRHKRAGHGAKNKLKPITMMTEKSKRFRKKLIERWACEIADFFIKNKVGTVQMENLESMKRKEDSYFNIRLRGFWPYAEMQDKIEFKLKQYGIVVRKVAPNNTSKTCSKCGHLNHYFNFEYRKKNKFPHFKCEKCNFKEDADYNAALNISNPKLKSTKGEP

SEQ ID NO: 1109 - protein, 726 aa, synthetic construct
SEVEFSHEYWMRHALTLAKRARDEHEVPVGAVLVLNNRVIGEGWNRAIGLHDPTAHAEIMALRQGGLVMQNYRLTDATLYVTFEPCVMCAGAMIHSRIGRVVFGVRNSKRGAAGSLMNVLNYPGMNHCVEITEGILVDECAALLCDFYRMPRQVLNAQKKAQSSISSGGSSGGSSGSETPGASESATPKSSGGSSASSTKNTITKTLKLRIVRPYNSAEVEKIVADEKNNRERIALEKNKDKVKEACSKHLKVAAYCTTQVERNACLFCKARKLDDKFYQKLRGQFPDAVFWQEIGEIFRQLQKQTAEIYNQSLIELYYEIFIKGKGFANASSVEHYLSDVCYTRAAELFKNAAIASGLRGKVKSNFRLKELKNMKSGLPTTKSDNFPIPLVKQKGGQYTGFEISSHNDDFIIKIPFGRWQVKKEIDKYRPWEKFDFVQVRKSPKPISLLLSTQRRKRNKGWSKDEGTEAEIRKVMNGDYQTSYIEVKRGSKIGEKSAWMLNLSIDVPKIDKGVDPSIIGGIDVGVRSPLVCAINNAFSRYSVSDNDLFRFNKKMFARRRILLKKNRHKRAGHGAKNKLKPISILTGKSERFRKKLIERWACEIADFFIKNKVGTVQMENLESMKRKEDSYFNIRLRGFWPYAEMQNKIEFKLKQYGIEIRKVAPNNTSKTCSKCGHLNNYFNFEYRKKNKFPHFKCEKCNFRENADYNAALNISNPKLKSTKEEP

SEQ ID NO: 1110 - protein, 726 aa, synthetic construct
SEVEFSHEYWMRHALTLAKRARDEREVPVGAVLVLNNRVIGVGWNRAIGLHDPTAHAEIMALRQGGLVMQNYRLVDATLYVTFEPCVMCAGAMVHSRIGRVVFGVRNGKRGAAGSLMNILDYPGMGHRVEITEGILADECAALLCDFYCMPRQVFNAQRRAQSSINSGGSSGGSSGSETPGTSESATPESSGGGSSGSAKNTITKTLQLRIVRPYNSAEVEKIVADEKNNREKIALEKNKDKVREACSKHLKVASYCTTQVERNACPFCKARKLDDKFYQKLRGQFPDAVFWQELGEIFRQLQKQAAEIYNQSLIELYYEIFIKGKGFANASSVEHYLSDVCYTRAAELFKNAAIASGLRGKVKSNFRLKELKNMKSGLPTTKSDNFPIPLVKQKGGQYTGFEISSHNDDFIIKIPFGRRQVKKEIDKYRPWEKFDFEQVRKSPKPISLLLSTQRRRRNKGWSKDEGTEAEIRKVMNGDYQTSYIEVKRGNKIGEKSAWMLNLSIDVPKIDKGVDPSIIGGIDVGVKSPLVCAINNALSRYSISDNDLFRFNKKMFARRRILLKKNRHKRAGHGAKNKLKPISILTGKGERFRKKLIERWACEIADFFIKNKVGTVQMENLESMKRKEDSYFNIRLRGFWPYAEMQNKIEFKLKQYGIEIRKVAPNNTSKTCSKCGHLNNYFNFEYRKKNKFPHFKCEKCNFKENADYNAALNISNPKLKSTKEEP

SEQ ID NO: 1111 - protein, 726 aa, synthetic construct
SEVEFSHEYWMRHALTLAKRARDEREVPVGAILVLNNRVIGEGWNRAIGLHDPTAHAEIMALRQGGLVTQNYRLIDATLYVTFEPCVMCAGAMIHSRIGRVVFGVRNSKHGAAGSLMNVLNYPGMNHRVEITEGILADECAALLCDFYRMPRQVFNARKKAQSSINPGGSSGGSSGSETLGTSESPTPESPGGSSGSSAKNTITKTLQLMIVRPYNSAEVEKIVADEKNNREKIALEKNKDKVKEACSKHLKVASYCTTQVERNACLFCKARKLDDKFYQRLRGQFPDAVFWQELGEIFRQLQKQAAEIYNQSLIELYYEIFIKGKGFANASSVEHYLSDVCYTRAAELFKNAAIASGLRGKVKSNFRLKELKSMKSGLPTTKSDNFPIPLVKQKGGQYTGFEISSHNSDFIIKIPFGRWQVKEEIDKYRPWEKFDFEQVRKSPKPISLLLSTQRRKRNKGWSKDEGTEAEIRKVMNGDYQTSYIEVKRGSKTGEKSTWMLNLSIDVPKIDKGVDPSIIGGIDVGVKSPLVCAINNAFSRYSISDNDLFRFNKKMFARRRILLGKNRHKRAGHGVKNKLKPITILTERSGRFRKKLIERWACEIADFFVKNKVGTVQMENLESMKRKEDSYFNIRLRGFWPYAEMQNKIEFKLKQYGIKVRKVAPNNTSKTCSKCGHLNNYFNFEYRKKNKFPHFKCEKCNFKENADYNAALNISDPKLKSTKEEH

SEQ ID NO: 1112 - protein, 726 aa, synthetic construct
SEVEFSHEYWMRHALALAKRARDEREVPVGAVLVLNNRAIGEGWNRAVGLHDPTAHAEIMALRQGGLVMQNYRLVEATLYVTFEPCIMCAGAMIHSRISRVVFGVRNSKRGAAGSLMNVLYYPGMNHRVEITEGILADECAALLCDYYRMPRQVFNAQKKAQSSISSGGPSGGSSCSETPGASESVTPKSSGGSSTGSTKNTITKTLKLRIVRPYNSAEVEKIVADEKNNREKIALEKNKDKVKEACSEHLKVAAYCTTQVERNACLFCKARKLDDRFYQKLRGQFPDAVFWQELGEIFRQLQKQAAEVYNQSLIELYYEIFIKGKGFANASSVEHYLSDVCYTRAAELFKNAAIASGLRGKVKSNFRLKELKNMKSGLPTTKSDNFPIPLVKQKGGQYTGFEISSHNDDFIIKIPFGRWQVKKEIDKYRPWEKFDFEQVRKSPKPISLLLSTQRRKRNKGWSKDEGTEAEIRKVMNGDYQTSYIEVKRGSKIGEKSAWMLSLSIDVPKIDKGVDPSIIGGIDVGVKSPLVCAINNAFCRYSISDNDLFHFNKKMFARRRILLKKSRHKRAGHGAKNKLKPISILTEKSKRFRKKLIERWACEIADFFIKNKVGTVQMENLESMKRKEDSYFNIRLRGFWPYAEMQNKIEFKLKQYGIEIRKVAPNNTSKTCSKCGHLNNYFNFEYRKKNKFPHFKCEKCNFKENADYNAALNISNPKLKSTKEEP

SEQ ID NO: 1113 - protein, 726 aa, synthetic construct
SEVEFSHEYWMRHALTLAKRARDEREVPVGAVLVLNNRVIGEGWNRAIGLHDPTAHAEIMALRQGGLVMRNYRLTDATLYVTFEPCVMCAGAMIHSRIGRVVFGVRNSKRGAAGSLMNVLNYPGMNHCVEITEGILVDECAALLCDFYRMPRQVLNAQKKAQSSISPGGSSGGSSDSETPGASESVIPKSSGGSSGGSAKNTITKTLKLRIVRPYNSAEVEKIVADEKNNRERIALEKNKGKVKEACSKHLEVAAYCTTQVERNACLFCKARKLDDKFYQKLRGQFPDAVFWQELGEIFRQLQKQAAEIYNQSLIELYYEIFIKGKGIANASSVEHYLSDVCYTRAAELFKNAAIASGLRNKVKSNFRLKELRSMKSGLPTTKSDNFPIPLVRQKGGQYTGFEISNHNSDFIIKIPFGRWQAKKEIDKYRPWEKFDFEQVRKSPKPISLLLSTQRRKRNKGWSKDEGTEAEIRKVMNGVYQTSYIEVKRGSKIGEKSAWMLNLSIDVPKIDKGADPSIIGGIDVGVKSPLVCAINNALSRYSISDNDLFHFNKKMFARRRILLRKNRHKRAGHGARNKLKPITVLTEKSERFRKKLIERWACEIANFFIKNKVGTVQMENLESMKRREDSYFNIRLRGFWPYAEMQSKIEFKLKQYGIEIRKVAPNNTSKTCSKCGHLNNYFNFEFRKKNKFPHFKCEKCNFKENADYNAALNISNPKLKSTKGEP

SEQ ID NO: 1114 - protein, 726 aa, synthetic construct
SEVEFSHEYWMRHALTLAKRARDEREVPVGAILVLNNRVIGEGWNRAIGLHDPTAHAEIMALRQGGLVMQNYRLIDATLYVTFEPCVMCAGAMIHSRIGRVVFGVRNSKHGAAGSLVNVLNYPGMNHRVEITEGILADECAALLCDFYRMPRQVFNARKEAQSSINSGGSSGGSSGSVTPGASGSVTPKSSGGSSAGSTKDTITKTLKLRIVRPYNSAEVEKIVADEKNNREKIALEKNKDKVKEACSKHLKVASYCTTQVERNACPFCKARKLDDKFYQKLRGQFPDAVFWQELGEILRQLQKQAAEIYNQSLIELYYEIFIKGKGFANASSVEHYLSDVCYSRAAELFKNAAIASGLRGKVKSNFRLKELKNMKSGLPTTKSDNFPIPLVKQKGGQYTGFEISSHNDDFIIKIPFGRWQVKKEIDRYRPWEKFDFEQVRKSPKPISLLLSTQRRKRNKGWSKDEGTEAEIKKVMNGDYQTSYIEVKRGSKTGEKSAWMLNLSIDVPKIDKGVDPSIIGGIDVGVKSPLVCAINNAFSRYSIGDNDLFHYNKKMFARRRILLRKNRHKRAGHGAKNKLKPITMMTEKSKRFRKKLIERWACEIADFFIKNKVGTVQMENLESMKRKEDSYFNIRLRGFWPYAEMQNKIEFKLKQYGIVVRKVAPNNTSKTCSKCGHLNNYFDFEYRKKNKFPHFKCEKCNFKEDADYNAALNISNPKLKSTKEEP

SEQ ID NO: 1115 - protein, 726 aa, synthetic construct
SEVEFSHEYWMRHALALAKRARDEREVPVGAVLVLNNRAIGEGWNRAIGLHDPTAHAEIMALRQGGLVMQNYRLTDATLYVTFEPCVMCAGAMIHSRIGRVVFGVRNSKRGAAGSLMNVLNYPGMNHCVEITEGILADECAALLCDFYRMPRQVFNARKKAQSSISLGGSSGGSSGSETPGTSESATPESSGGSSGGSAKNTITKTLKLRIVRPYNSAEVEKIVADEKNSREKIALEKNKDKVKEACSKHLKVAAYCTTQVERNACLFCKARKLDDKFYQKLRGQFPDAVFWQEIGEVFRQLQKQAAEIYNQSLIELYYEIFIKGKGFANASSVEHYLSDVCYTRAAELFKNAAIASGLRGKVKSNFRLKELKNMKSGLPTTKSDNFPIPLVKQKGGQYTGFEISSHNDDFIIKIPFGRWQAKKEIDKYRPWEKFDFEQVRKSPKPISLLLSTQRRKRNKGWSKDEGTEAEIRKVMNGDYQTSYIEVKRGSKIGEKSAWMLNLSIDVPKIDKGVDPSIIGGIDVGVKSPLVCAINNAFSRYSIGDNDLFHYNKKMFARRRILLKKNRHKRAGHGAKNKLKPISILTEKSKRFRKKLIERWACEIADFFIRNKVGTVQIENLESMKRKEDSYFNIRLRGFWPYAEMQNKIEFKLKQYGIEIRKVAPNNTSKTCSKCGHLNSYFNFEYRKKNKFPHFKCEKCNFKENADYNAALNISNPKLKSTKEKP

SEQ ID NO: 1116 - protein, 726 aa, synthetic construct
SEVEFSHEYWMRHALTLAKRARDEREVPVGAVLVLNNRVIGEGWNRAIGLHDPTAHAEIMALRQGGLVMQNYRLTDATLYVTFEPCVMCAGAMIHSRIGRVVFGVRNSKRGAAGSLMNVLNYPGMNHCVEITEGILVDECAALLCDFYRMPRRVLNAQKKAQSNINPGGSSGGSSGSETPGTSESATLENSGGSSGGSAKNTITKTLKLRIVRPYNSAEVEKIVADEKNNRERVALEKNKDKVKEACSEHLRVAAYCTTQVERNACLFCKARKLDDKFYQKLRGQFPDAVFWQEIGEIFRQLQKQAAEIYNQSLIELYYEIFIKGRGFANASSVEHYLSDVCYTRAAELFKNAAIASGLRNKIKSNFRLKELRNMKSGLPTTKSDNFPIPLVKQKGGQYTGFEISNHNSDFIIKIPFGRWQAKKEIDKYRPWEKFDFEQVRKSPKPISLLLSTQRRKRNRGWSKDEGTEAEIKKVMNGDYQTSYIEVKRGSKIGEKSAWMLNLSIDVPKIDKGVDPSIIGGIDVGVKSPLVCAINNAFSRYSISDNDLFHFNKKMFARRRILLKKSKHKRAGHGAKNKLKPITIMTEKSKRFRKKLIERWACEIADFFIKNKVGTVQMENLESMKRKEDSYFNVRLRGFWPYAEMQNKIEFKLKQYGIVVRKVAPNNTSKTCSKCGHLNNYFNFEYRKKNKFPHFKCEKCDFKENADYNAALNISNPKLKNTKGEP

SEQ ID NO: 1117 - protein, 726 aa, synthetic construct
SEVEFSHEYWMRHALTLAKRARDEREVPVGAVLVLNNRVIGEGWNRAIGQHDPTAHAEIMALRQGGLVMQNYRLIGATLYVTFEPCVMCAGAMIHSRIGRVVYGVRNGKRGAAGSLMNVLNYPGMNHRVEITEGILADECAALLCDFYRMPRRVLNAQKRAQSSINSGGPSGGSSGSETPGTSESATPESPGGSSGGSAKNTITKTLKLRIVRPYNSAEVEKIVADEKNNREKIALEKNKDKVKEACSEHLKVAAYCTTQVERSACLFCKARKLDDKFYQKLRGQFPDAVFWQEIGEVFRQLQKQAAEIYNQSLIELYYEIFIKGKGFANASSVEHYLSDVCYARAAELFKNAAIASGLRGKVKSNFRLKELKNMKSGLPTTKSDNFPIPLVKQKGGQYTGFEISSHNDDFIIKIPFGRWQVKKEINKFRPWEKFDFEQVRKSPKPISLLLSTQRRKRNKGWSKDEGTEAEIRKVMNGDYQTSYIEVKRGSKIGEKSAWMLNLSIDVPKIDKGVDPSIIGGIDVGVKSPLVCAINNAFSRYSISDNDLFHFNKKMFARRRILLKKNRHKRAGHGAKNKLKPISILTEKGERFRKKLIEKWACEIADFFIKNKVGTVQMENLESMKRKEDSYFNIRLRGFWPYAEMQNKIEFKLKQYGIEIRKVAPNNTSKTCSKCGHLNNYFNFEYRKKNRFPHFKCEKCNFKENADYNAALNISNPELKSTKEEP

SEQ ID NO: 1118 - protein, 726 aa, synthetic construct
SEVEFSHEYWMRHALTLAKRARDEREVPVGAVLVLNNRVIGEGWNRAIGLHDPTAHAEIMALRQGGLVMQNYRLTDATLYVTFEPCVMCAGAMIHSRIGRVVFGVRNSKRGAAGSRMNVLNYPGMNHCVEITEGILVDECAALLCDFYRMPRQVLNAQKKTQSSISSGGSSGGSSGSETPGASGSVIPKSSGGSSAGSTKDTITKTLKLRIVRPYNSAEVEKVVADEKNNREKIAMEKNKDKVKEACSKHLKVATYCTTQVERNACLFCKARKLDDKFYQKLRGQFPDAVFWQEIGEIFRQLQKQAAEIYNQSLVELYYEIFIKGKGIANASSVEHYLSDVCYTRAAELFKNAAIASGLRNKIKSNFRLKELRNMKSGLPTTKSDNFPIPLVRQKGGQYTGFEISNHNGDFIIKIPFGRWQVKKEISKHRPWEKFDFEQVRKSPKPISLLLSTQRRKRNRGWSKDEGTEAEIRKVMNGDYQTSYIEVKRGSKIGEKSAWMLNLSIDVPKIDKGVDPSIIGGIDVGVKSPLVCAINNASSRYSISDNDLYHFNKKMFARRRILLKKNRHRRAGHGAKNKLKPITTLTEKSGRFRKKLIERWACEIANFFIKNEVGTVQMENLESMKRKEDSYFNIRLRGFWPYAEMQNKIEFKLKQYGIKIRKVAPNNTSRTCSKCGHLNNYFSFEYRKKNKFPHFKCEKCNFKEDADYNAALNISNPKLKGTKEEL

SEQ ID NO: 1119 - protein, 726 aa, synthetic construct
SEVEFSHEYWMRHALSLAKRARDEREVPVGAVLVLNNRIIGVGWNRAIGLHDPTAHAEIMALRQGGLVMQNYRLVDATLYVTFEPCVLCAGAMVHSRIGRVVFGVRNSKRGAAGSLMNVLNHPGMNHRVEITGGILADECAALLCDFYRMPRQVFNAQKKARSNINSGGSSGGSSGSETLGTSESATPESSGGSSGGSAKNTITKTLKLRIVRPYNSAEVEKIVADEKNNREKIALEKNKDKVKEACSEHLKVAAYCTTQVERNACLFCKARKLDDKFYQKLRGQFPDAVFWQEIGEIFRQLQRQAAEIYNQSLIELYYEIFIKGKGFANASSVEHYLSDVCYTRAAELFKNAAIASGLRGKVKSNFRLKELKNMKSGLPTTKSDNFPIPLVKQKGGQYTGFEISSHNDDFIIKIPFGRWQVKKEIDKYRPWEKFDFEQVRKSPKPISLLLSTQRRKRNKGWSKDEGTEAEIRRVMNGDYQTSYIEVKRGSKIGEKSAWMLNLSIDVPKIDKGVDPSIIGGIDVGVKSPLVCAINNAFSRYSISDNDLFRFNKKMFARRRILLKKNRHKRAGHGAKNKLKPISILTGKSERFRKKLIERWACEIADFFIKNKVGTVQMENLESMKRKEDSYFNIRLRGFWPYAEMQNKIEFKLKQYGIEIRKVAPNNTSKTCSKCGHLNNYFNFEYRKMNKFPHFKCEKCNFKENADYNAALNISNPKLKSTKEEP

SEQ ID NO: 1120 - protein, 726 aa, synthetic construct
SEVEFSHEYWMRHALTLAKRARDEREVPVGAVLVLNNRVIGEGWNRTTGLHDPTAHAEIMALRQGGLVMQNYRLTDATLYVTFEPCVMCAGAMVHSRIGRVVFGVRNSKRGAAGSLMNVLNYPGMSHCVEITEGILVDECAALLCDFYRMPRQVLNAQKKAQSSISSGGSSGGSGGGETPGASESVTPKSSGGSSDGSAKNTITKTLKLRIVRPYNSAEVEKIVADEKNNREKIALEKNKDKVREACSKHLKVAAYCTTQVERNACLFCKARKLDDKFYQKLRGQFPDAVFWQETGEIFRQLQKQAAEIYNQSLIELYYEIFIKGKGFANASSVEHYLSDVCYTRAAELFKNAAIASGLRGKVKSNFRLKELKNMKSGLPTTKSDNFPIPLVKQKGGQYTGFEISSHNDDFIIKIPFGRWQVKKEIDKYRPWEKFDFEQVRKSPKPISLLLSTQRRKRNKGWSKDEGTEAEIRKVMNGDYQTSYIEVKRGSKIGEKSAWMLNLSIDVPKIDKGVDPSIIGGIDVGVKSPLVCAINNALSRYSISDNDLFHFNKKMFARRRILLKKNRHKRAGHGARNKLKPITVLTEKSERFRKKLIERWACEIAYFFIKNKVGTVQMEDLESMKRKEDSYFNIRLRGFWPYAEMQNKIEFKLKQYGIKIRKVAPNNTSRTCSKCGHLNNYFSFEYRKKNKFPHFKCEKCNFKEDADYNAALNISNPKLKSTKEEP

SEQ ID NO: 1121 - protein, 726 aa, synthetic construct
SEVEFSHEYWMRHALTLAKRARDEREVPVGAVLVLNDRAIGEGWNRAIGLHDPTAHAEIMALRQGGLVMQNYRLIDATLYVTFEPCAMCAGAMVHSRIGRVVFGVRNSKRGAAGSLMNVLNYPGMDHRVEITGGILADECAALLCDFYRMPRQVFNARKKTQSSINPGGSSGGSSGSETPGTSESATPESSGGSSGSSAKNTITKTLKLRIVRPYNSAEVEKIVADEKNNREKIALEKNKDKVKEACSKHLKVAAYCTTQVERNACLFCKARRLDDKFYQKLRGQFPDAVFWQEIGEIFRQLQKQAAEVYNQSLVELYYEILIKGKGIANASSVEHYLSDVCYTRAAELFKNAAIASGLRNKIKSNFRLKELRNMKSGLPTTKSDNFPIPLVRQKGGQYTGFEISNHDGDFIIKIPFGRWQVKKEINKHRPWEKFDFEQVRKSPKPISLLLSTQRRKRNKGWSKDEGTEAEIRRVMNGDYQTSYIEVKRGSKIGEKSAWMLNLSIDVPKIDKGVDPSIIGGIDVGVKSPLVCAINNALSRYSISDNDLFHFNKKMFARRRILLRKNRHKRAGHGAKNKLKPITIMTEKSKRFRKKLIERWACEIADFFIKNKVGTVQMENLESMKRKEDSYFNIRLRGFWPYAEMQNKIEFKLKQYGIKIRKVAPNNTSRTCSKCGHLNNYFSFEYRKKNKFPHFKCEKCNFKEDADYNAALNISNPKLKGTKEEL

SEQ ID NO: 1122 - protein, 726 aa, synthetic construct
SEVEFSHEYWMRHALTLAKRARDEREVPVGAILVLNNRVVGEGWNRAIGLHDPTAHAEIMALRQGGLVMQNYRLIDATLYVTFEPCVMCAGAMIHSRIGRVVFGVRNSKHGAAGSLMDVLNYPGMNHRVEITEGILADECAALLCDFYRMPRQVFSARRKAQSSINPGGSSGGSSGSETPGASESVTPKSSGGSSGGSAKNTITKTLKLRIVRPYNSAEVEKIVADEKNNREKIALEKNKGKVKEACSKHLEVAAYCTTQVERNACLFCKARKLDDKFYQRLRGRFPDAVFWQELGEIFRQLQKQAAEIYNQSLIELYYEIFIKGKGFANASSVEHYLSDVCYTRAAELFKNAAIASGLRGKVKSNFRLKELRNMKSGLPTTKSDNFPIPLVKQKGGQYTGFEISSHNDDFIIKIPFGRWQEKEEIGKYRPWEKFDFEQVRRSPKPISLLLSTQRRKKNKGWSKDEGTEAEIRRVMNGDYQTSYIEVKRGSKIGEKSAWMLNLSIDVPKIDKGVDPSIIGGIDVGVKSPLVCAINNAFSRYSISDNDLFHFNKKMFARRRILLKKNRRRRAGHGAKNKLKPITILTEKSVRFRKKLIERWACEIADFFIKNKVGTVQMENLESMKRKEDSYFNIRLRGFWPYAEMQNKIEFKLKQYGIEIRRVAPNNTSRTCSKCGHLNNYFNFEYRRKYKFPHFKCEKCNFKEDADYNAALNISNPKLKSTKEEP

SEQ ID NO: 1123 - protein, 726 aa, synthetic construct
SEVEFSHEYWMRHALALAKRARDEREVPVGAILVLNNRVIGEGWNRAIGLHDPTAHAEIMALRQGGLVMQNYRLIDATLYVTFEPCVMCAGAMIHSRIGRVVFGVRNNKHGAAGSLVNVLNYPGMNHRVEITEGILADECAALLCDFYRMPRQVFNARKKAQSSISPGGSSGGSSGSETPGTSESAAPESSGGSSGGSTKNTITKTLKLRIVRPYNSAEVEKIVADEKNSREKIALERNKDKVKEACSEHLKVAAYCTTQVERNACLFCKARKLDDRFYQKLRGQFPDAVFWQETGEIFRQLQRQAAEIYNQSLIELYYEIFIKGKGFANASSVEHYLSDVCYTRAAELFKNAAIASGLRGKVKSNFRLKELRNMKSGLPTTKSDNFPIPLVKQKGGQYTGFEISSHNDDFIIKIPFGRWQVKKEIDKYRPWEKFDFEQVRKSPKPISLLLSTQRRKRNKGWSKDEGTEAEIRKVMNGDYQTSYIEVKRGSKTGEKSAWMLNLSIDVPKIDKGVDPSIIGGIDVGVKFPLVCAINNAFSRYSISDNDLFRFNKKMFARRRILLKKNRHKRAGHGAKNKLKPISILTGKSERFRRKLIERWACEIADFFIKNKVGTVQMENLESMKRKEDSYFNIRLRGFWPYAEMQNKIEFKLKQYGIKIRKVAPNNTSRTCSKCGHLNNYFSFEYRKKNKFPHFKCEKCNFKEDADYNAALNISNPKLKGTKEEL

SEQ ID NO: 1124 - protein, 726 aa, synthetic construct
SEVEFSHEYWMRHALTLAKRARDEREVPVGAVLVLNNRVIGEGWNRAIGLHDPTAHAEIMALRQGGLVMQNYRLIDATLYVTFEPCVMCAGAMIHSRVGRVVFGVRNSKHGAAGSLMNVLNYPGMNHRVEITEGILADECAALLCDFYRMPRRVFNARKKAQSSIDPGGPSGGSSGNETPGTSESATPESSGGSSGGSAKNTITKTLKLRIVRPYNSTEVEKIVADEKNNREKVALEKNKDKVKEACSKHLKVASYCTTQVERNACLFCKARKLDDKFYQKLRGQFPDAVFWQELGEIFRQLQKQAAEIYNQSLIELYYEIFIKGKGFANASSVEHYLSDVCYTRAAELFKNAAIASGLRGKVKSNFRLKELKNMKSGLPTTKSDNFPIPLVKQKGGQYTGFEISSHNDDFIIKIPFGRWQVKKEIDKYRPWEKFDFEQVRKSPKPISLLLSTQRRKRNKGWSKDEGTEAEIRKVMNGDYQTSYIEVKRGSKIGEKSAWMLNLSIDVPKIDKGVDPSIIGGIDVGVKSPLVCAINNAFSRYSISDNDLFHHNKKMFARRRILLKKNRHKRAGHGAKDKLKPISILTEKSKRFRKKLIERWACEIADFFIKNKVGTVQMENLESMKRKEDSYFNIRLRGFWPYAEMQNKIEFKLKQYGIEIRKVAPNNTSKTCSKCGHLNNYFNFEYRKMNKFPHFKCEKCNFKENADYNAALNISNPKLKSTKEEP

SEQ ID NO: 1125 - protein, 726 aa, synthetic construct
GEDEFSHEYWMRHALTLAKRARDGREVPVGAVLVLNNRVIGEGWNRAIGLHDPTAHAEIMALRQGGLVMQNYRLIDATLYVTFEPCVMCAGAMVHSRIGRVVFGVRNSKRGAAGSLMNVLDYPGMGHRVEITEGILVDECAALLCDFYRMPRRVLNAQKKAQSSISSGGSSGGCSGSEMSGASESVTPKSSGGSSAGSTKNTITKTLKLRIVRPYNSAEVEKIVADEKNSREKIALERNKDKVKEACSEHLKVAAYCTTQVERNACLFCKARKLDDRFYQKLRGQFPDAVFWQETGEIFRQLQRQAAEIYNQSLIELYYEIFIKGKGFANASSVEHYLSDVCYTRAAELFKNAAIASGLRGKVKSNFRLKELKNMKSGLPTTKSDNFPIPLVKQKGGQYTGFEISSHNDDFIIKIPFGRWQVKKEIDKYRPWEKFDFEQVRKSPKPISLLLSTQRRKRNKGWSRDEGTEAEIRKVMNGDYQTSYIEVKRGSKIGEKSAWMLSLSIDVPKIDKGVDPSIIGGIDVGVKSPLVCAINNAFCRYSISDNDLFHFNKKMFARRRILLKKSKHKRAGHGAKNKLKPITILTEKSGRFRKKLIERWACEIADFFIKNKVGTVQMENLEGMKRKEDSYFNIRLRGFWPYAEMQNKIEFKLKQYGIEIRKVAPNNTSKTCSKCGHLNSYFNFEYRKKNKFPHFKCEKCNFKEDADYNAALNISNPKLKSTKEEP

SEQ ID NO: 1126 - protein, 726 aa, synthetic construct
SEVEFSHEYWMRHALTLAKRARDEREVPVGAVLVLNNRVIGEGWNRTTGLHDPTAHAEIMALRQGGLVMQNHRLVDATLYVTFEPCVMCAGAMIHSRIGRVVFGVRNSKRGAAGSLMNVLNYPGMNHCVEITEGILVDECAALLCDFYRMPCQVLNAQKKAQSSISSGGSSGGSSGSDTLGASESVTPKSSVGSSASSTKNTITKTLKLRIVRPYNSAEVEKIVADEKDNREKIALEKNKDKVKEACSKHLKVAAYCTTQVERNACLFCKARRLDDKFYQKLRGQFPDAVFWQEIGEIFRQLQKQAAEIYNQSLIELYYEIFIKGKGFANASSVEHYLSDVCYTRAAELFKNAAIASGLRGKVKSNFRLKELKNMRSGLPTTKSDNFPIPLVKQKGGQYTGFEISSHSDDFIIKIPFGRWQVKKEIDKYRPWEKFDFEQVRKSPKPISLLLSTQRRKRNRGWSKDEGTEAEIRKVMNGDYQTSYIEVKRGSKIGEKSAWMLNLSIDVPKIDKGVDPSIIGGIDVGVKSPLVCAINNAFSRYSISDNELFHFNKKMFARRRILLKKNRHRRAGHGAKNKLKPITILTEKSKRFRKKLIERWACEIADFFIKNKVGTVQMENLESMKKKEDSYFNIRLRGFWPYAEMQNKIEFKLKQYGIEIRKVAPNNTSRTCSKCGHLNNYFNFEYRKKNKFPHFKCEKCNFKEDADYNAALNISNPKLKSTKEEH

SEQ ID NO: 1127 - protein, 726 aa, synthetic construct
SEVEFSHEYWMRHALSLAKRARDEREVPVGAVLVLNNRVIGEGWNRAIGLHDPTAHAEIMALHQGGLVMQNYRLIDATLYVTFEPCVMCAGAMIHSRIGRVVFGARNSKRGAAGSLMNVLSYPGMNHRVEITEGILADECAALLCDFYRMPRRVFNAQKKAQSSINSGGSSGGGSGSDTPSTSESTTPESSGGSSGGPAKNTVTKTLKLRIVRPYNSAEVEKIVADEKNNREKTALEKNKDKVKEACSKHLKVAAYCTTQVERNACLFCKARKLDDKFYQKLRGQFPDAVFWQEVGGIFRQLQKQAAEVYNQSLIELYYEIFIKGKGFANASSVEHYLSDVCYTRAAELFKNAAIASGLRGKVKSNFRLKELKNMKSGLPTTKSDNFPIPLVKQKGGQYTGFEISSHNDDFIIKIPFGRWQVKKEIDKYRPWEKFDFEQVRKSPKPISLLLSTQRRRRNKGWSKDEGTEAEIRKVMNGDYQTSYIEVKRGSKIGEKSAWMLSLSIDVPKIDKGVDPSIIGGIDVGVKSPLVCAINNAFCRYSISDNDLFHFNKKMFARRRILLKKSRHKRAGHGAKNKLKPISILTEKSKRFRKKLIERWACEIADFFIKNKVGTVQMENLESMKRKEDSYFNIRLRGFWPYAEMQNKIEFKLKQYGIVIRKVAPNNTSKTCSKCGHLNNYFNFEYRKKNKFPHFKCEKCNFKENADYNAALNISNPKLKSTKEEP

SEQ ID NO: 1128 - protein, 726 aa, synthetic construct
SEVEFSHEYWMRHALTLAKRARDEREVPVGAVLVLNNRVIGEGWNRTTGLHDPTAHAEIMALRQGGLVMRNYRLTDATLYVTFEPCVMCAGAMIHSRIGRVVFGVRNSRRGAAGSLMNVLNYPGMNHCVEITEGILVDECAALLCDFYRMPRQVLNAQKKAQSSISPGGSSGGSSGSETPGASESVTPKSSGGSSGGSAKNTITKTLKLRIVRPYNSAEVEKIVADEKNNREKIALEKNKDKVREACSKHLKVASYCTTQVERNACPFCKARKLDDKFYQKLRGQFPDAVFWQELGEILRQLQKQAAEIYNQSLIELYYEIFIKGRGFANASSVEHYLSDVCYTRAAELFKNAAIASGLRGKVKGNFRPKELKNMKSGLPTTKSDNFPIPLVKQKGGQYTGFEISSHNDDFIIKIPFGRWQVKKEVDKYRPWEKFDFEQVRKSPKPISLLLSTQRRKRNKGWIKDEGTEAEIRKVMNGDYQTSYIEVKRGSKIGEKSAWMLNLSIDVPKIDKGVDPSIIGGIDVGVKSPLVCAINNAFSRYSISDNDLFHFNKKVFARRRILLKKNRHKRTGHGARNKLKPITVLAEKSERFRKKLIERWACEIANFFIKNKVGTVQMENLESMKRKEDSYFNIRLRGFWPYAEMQNKIEFKLKQYGIEIRKVAPNNTSKTCSMCGHLNNYFNFEYRKRNKFPHFKCEKCNFKENADYNAALNISNPKLKSTKEEP

SEQ ID NO: 1129 - protein, 726 aa, synthetic construct
SEVEFSHEYWMRYALTLAKRARDEREVPVGAVLVLNNRVIGEGWNRAIGLHDPTAHAEIMALRQGGLVMQNYRLTDATLYVTFEPCVMCAGAMIHSRIGRVVFGVRNSKRGAAGSLMNVLNYPGMNHCVEITEGILMDECAALLCDFYRMPRQVLNAQKKAQSSISSGGPSGGSSCSETPGASESVTPKSSGGSSTGSTKNTITKTLKLRIVRPYNSAEVEKIVADEKNSREKIALEKNKDKVKEACSEHLKVAAYCTTQVERNACLFCKARKLDDKFYQKLRGQFPDAVFWQEIGEIFRQLQKQAAEIYNQSLIELYYEIFIKGRGFANASSVEHYLSDVCYTRAAELFKNAAIASGLRGKVKSNFRLKELKNMKSGLPTTKSDNFPIPLVKQKGGQYTGFEISSHNDDFIIKIPFGRWQVKEEIDKYRPWEKFDFEQVRKSPKPISLLLSTQGRQKNKGWSKDEGTEAEIRRVMNGDYQTSYIEVKRGSKIGGKSTWMLNLSIDVPKIDKGVDPSIIGGIDVGVKSPLVCAINDALSRYSISDNDLFHFNKKMFARRRILLKKNRHKRAGHGAKNKLKPISILTEKSERFRKKLIERWACEIADFFIRNKVGTVQMENLEGMKRKEDSYFNIRLRGFWPYAEMQNKIEFKLKQYGIEIRKVAPNNTSKTCSKCGHLNNYFNFEYRKKNKFPHFKCEKCNFKENADYNAALNISNPKLKSTKEGP

SEQ ID NO: 1130 - protein, 726 aa, synthetic construct
SEVEFSHEYWMRHALTLAKRARDEREVPVGAVLVLNNRVIGEGWNRAIGLHDPTAHAEIMALRQGGLVMQNYRLIDATLYVTFEPCVMCAGAMIHSRIGRVVFGVRNNKHGAAGSLVNVLNYPGMNHRVEITEGVLADECAALLCDFYRMPRQVFNARKKAQSSINPGGSSGGSGGSETPGTSESATPESSGGSSGSSAKNTITKTLKLRIVRPYNSAEVEKIVADEKNNREKIALEKNKDKVKEACSKHLKVAAYCTTQVERNACLFCKARKLDDKFYQKLRGRFPDAVFWQEIGEIFRQLQKQAAEIYNQSLIELYYEIFIKGKGFANASSVEHYLSDVCYTRAAELFKNAAIASGLRGKVKSNFRLKELKNMKSGLPTTKSDNFPIPLVKQKGGQYTGFEISSHNDDFVIKIPFGRWQVKEEIDKYRPWEKFDFEQVRKNPKPISLLLSTQRRKRNKGWSKDEGTEAEIRKVMNGDYQTSYIEVKRGSKIGEKSAWMLNLSIDVPKIDKGVDPGIIGGIDVGVKSPLVCAINNASSRYSISDNDLFHFNKKMFARRRILLKKNRHKRAGHGAKNKLKPITIMTEKSKRFRKKLIERWACEIADFFIKNKVGTVQMENLESMKRKEDSYFNIRLRGFWPYAEMQNKIEFKLKQYGIEIRKVAPNNTSKTCSKCGHLNNYFSFEYRKKNKFPHFKCEKCNFKEDADYNAALNISNPKLKSTKEEL

SEQ ID NO: 1131 - protein, 726 aa, synthetic construct
SEVEFSHEYWMRHALTLAKRARDEREVPVGAVLVLNNRVIGEGWNRAIGLHDPTAHAEIMALRQGGLVMQNYRLTDATLYVTFEPCVMCAGAMIHSRIGRVVFGVRNSKRGAAGSLMNVLNYPGMNHCVEITEGILVDECAALLCDFYRMPRQVLNAQKKAQSSISSGGSSGGSGCSETPGASESVTPKSSGGSSAGSTKNTITKTLKLRIVRPYNSAEVEKIVADEKNSRERIALEKNKDKVKEACSEHLKVAAYCTTQVERSACLFCKARKLDDGFYQKLRGQFPDAVFWQEIGEIFRQLQKQAAEIYNQSLIELYYEIFIKGKGFANASSVEHYLSDVCYTRAAELFKNAAIASGLRGKVKSNFRLKELKNMKSGLPTTKSDNFPIPLVKQKGGQYTGFEISSHNDDLIVKIPFGRWQVKKEIDRYRPWEKFDFEQVRKSPKPISLLLSTQRRKRNKGWSKDEGTEAEIRKVMSGDYQTSYIEVKRGSKIGEKNAWMLNLSIDVPKIDKGVDPGIIGGIDVGVKSPLVCAINNAFSRYSISDNDLFRFNKKMFARRRILLKKNRYKRAGHGAKNKLKPITILTKKSERFRKKLIERWACEIADFFIKNKVGTVQMENLESMKRKEDSYFNVRLRGFWPYAEMQNKIEFKLKQYGIEIRKVAPNNTSKTCSKCGHLNNYFNFGYRKRNKFPHFKCEKCNFKEDADYNAALNISNPKLKSTKEEP

SEQ ID NO: 1132 - protein, 726 aa, synthetic construct
SEVEFSHEYWMRHALTLAKRARDEREVPVGAILVLNNRVIGEGWNRAIGLHDPTAHAEIMALRQGGLVMQNYRLIDATLYVTFEPCVMCAGAMVHSRIGRVVFGVRNSKRGAAGSLMNVLDYPGMGHRVEITEGILADECAALLCDFYCMPRQVFNAQKRAQSSVSSGGSSGGSSGGETPGASERATPKSSGGSSGGSTKNTITKTLKLRIVRPYNSAEVEKIVADEKNNRERIALEKNKDKVKEACSKHLKVAAYCTTQVERNACLFCKARRLDDKFYQKLRGQFPDAVFWQEIGEIFRQLQKQAAEIYNQSLVELYYEIFIKSKGIANASSVEHYLSDVCYTRAAELFKNAAIASGLRNKIKSNFRLKELKSMKSGLPTTRSDNFPIPLVKQKGGQYTGFEVSSHNDDFIIKIPFGRWQVKKEIDKYRPWEKFDFEQVRKSPKPISLLLSTQRRKRNKGWSKDEGTEAEIRKVMNGDYQTSYIEVKRGSKTGEKSAWMLNLSIDVPKIDKGVDPSIIGGIDVGVKSPLVCAINNALSRYSISDNDLFRFNKKMFARRRILLKKNRHKRAGHGAKNKLKPISILTRKSERFRKKLIERWACEIADFFVKNKVGTVQMENLESMKRKEDSYFNIRLRGFWPYAEMQNKIEFKLKQYGIEIRKVAPNNTSKTCSKCGHLNSYFSFEYRKKNKFPHFKCEKCNFKENADYNAALNISNPRLKSTKEEP

SEQ ID NO: 1133 - protein, 726 aa, synthetic construct
SEVEFSHEYWMRHALTLAKRARDEREVPVGAVLVLNNRVIGEGWNRAIGLYDPTAHAEIMALRQGGLVMQNYRLSDATLYVTFEPCVMCAGAMIHSRIGRVVFGVRNSKRGAAGSLMNVLNYPGMNHCVEITEGILADECAALLCDFYRMPRQVFTAQKKARSNINSGGSSGGSSGSETPGTSESATPEGSGGSSGGSAKNTITKTLKLRIVRPYNSAEVEKIVADEKNNREKTALEKNKDKVKEACSEHLKVATYCTTQVERNACLFCKARKLDDKFYQRLRGQFPDAVFWQELGEIFRQLQKQAAEIYNQSLIELYYEIFIKGKGFANASSVEHYLSDVCYTRAAELFKNAAIASGLRGKVKSNFRLKELKNMKSGLPTTKSDNFPIPLVRQKGGQYTGFEISSHNDDFIIKIPFGRWQVRKEIDKYRPWEKFDFEQVRKSPKPISLLLSTQRRRRNKGWSKDEGTEAEIRKVMSGDYQTSYIEVKRGSKIGEKSAWMLNLSIDVPKIDKGVDPSIIGGVDVGVKSPLVCAINNAFSRYSISDNDLFRFNKKMFARRRILLKKNRHKRAGHGAKNKLKPISILTGKSERFRKKLIERWACEIADFFIKNKVGTVQMENLESMKRKEDSYFNIRLRGFWPYAEMQNKIEFKLKQYGIEIRKVAPDNTSKTCSKCGHLNNYFNFEYRKKNKFPHFKCEKCNFKENADYNAALNISNPRLKSTKEEP

SEQ ID NO: 1134 - protein, 726 aa, synthetic construct
SEVEFSHEYWMRHALTLAKRARDEREVPVGAVLVLNNRVIGVGWNRAIGLHDPTAHAEIMALRQGGLVMQNYRLIDATLYVTFEPCIMCAGAMIHSRIGRVVFGVRNSKRGAAGSLMNVLNYPGMNHRVEITEGVLADECAALLCDFYRMPRQVLNAQKKAQSSINSGGSSGGDSGGETPGTSESATQESSGGSSGGSAKNTITKTLKLRIVRPYNSAEVEKIVADEKNNREKIALEKNKDKVKEACSKHLKVAAYCTTQVERNACLFCKARKLDDKFYQKLRGQFPDAVFWQELGEILRQLQKQAAEIYNQSLIELYYEIFIKGKGITNASRVEHYLSDVCYTRAAELFKNAAIASGLRSKVRSNFRLKELKNMKSGLPTTRSDNFPIPLVKQKGGQYTGFEISSHNSDFIIKIPFGRWQVKEEIDKYRPWEKFDFEQVRKSPKPISLLLSTQRRKKNKGWSKDEGTEAEIRRVMNGDYQTSYIEVKRGSKIGEKSAWMLNLSIDVPKIDKGVDPSIIGGIDVGVKSPLVCAINNSSSRYSICDNDLFRFNKKMFARRRILLKKNRRRRAGHGAKNKLKPITILTEKSVRFRKKLIERWACEIADFFIKNKVGTVQMENLESMKRKEDSYFNIRLRGFWPYAEMQNKIEFKLKQYGIEIRRVAPNNTSRTCSKCGHLNNYFNFEYRKKNKFPHFKCEKCSFKENADYNAALNISNPKLKSTKGEP

SEQ ID NO: 1135 - protein, 726 aa, synthetic construct
SEVEFSHEYWMRHALTLAKRARDECEVPVGAILVLNNRVIGEGWNRAIGLHDPTAHAEIMALRQGGLVMQNYRLIDATLYVTFEPCVMCAGAMIHSRIGRVVFGVRNSKYGAAGSLVNVLNYPGMNHRVEITEGILADECAALLCDFYRMPRQVFNARKKAQSSINPSGSSGGSSGSVTPGTSESATPESSGGGFGGSAKNTITKTLQLRIVRPYNSAEVEKIVADEKNNREKIALEKNKDKVKEACSKHLKVASYCTTQVERNACLFCKARKLDDKFYQKLRGQFPDAVFWQELGEIFRQLQKQAAEIYNQSLIELYYEIFIKGKGLANASSVEHYLSDVCYTRAAESFKNAAIASGLRGKVKSNFRLKELKNMKSGLPTTKSDNFPIPLVKQKGGQYTGFEISSHNDDFIIKIPFGRWQVKKEIDKYRPWEKFDFEQVRKSPKPISLLLSTQRRKRNKGWSKDEGTEAEIRKVMNGDYQTSYIEVKRGSKIGEKSAWMLNLSIDVPKIDKGVDPSIIGGIDVGVKSPLVCAINNAFSRYSISDNDLFHFNKKMFARRRILLKKNRHKRAGHGAKNKLKPITILTEKSGRFRKKLIERWACEIADFFIKNKVGTVQMENLESMKRKEDSYFNIRLRGFWPYAEMQNKIELKLKQYGIKIRKVAPNNTSKTCSKCGHLNDYFNFEYRKKNKFPHFKCEKCNFKEDADYNAALNISNPKLKSTREEP

SEQ ID NO: 1136 - protein, 726 aa, synthetic construct
SEVEFSHEYWMRHALTLAKRARDEREVPVGAILVLNNRVIGVGWNRAIGLHDPTAHAEIMALRQGGLVMQNYRLIDATLYVTFEPCVMCAGAMIHSRIGRVVFGVRNGKHGAAGSLMNALNYPGMNHRVEITEGILADECAALLCDFYRMPRQVFNGRKKAQSSINSGGSSGGSSGSETPGTSESATPESSGGSSGGSAKNTITKTLKLRIVRPYNSAEVEKIVADEKNNRERIALEKNKDKVKEACSKHLKVAAYCTTQVERNACLFCKARKLDDKFYQKLRDQFPDAVFWQEIGEIFRQLQRQAAEIYNQSLIELYYEIFIKGKGFANASSVEHYLSNVCYTRAAELFKNAAIASGLRGKIKSNFRLKELKNMKSGLPTTKSDNFPIPLVKQKGGQYTGFEISSHNDDFIIKIPFGRWQVKKEIDKYRPWEKFDFEQVRKSPKPISLLLSTQRRKRNKGWSKDEGTEAEIRKVMNGDYQTSYIEVKRGSKVGEKSAWMLNLSIDVPKIDKGVDPSIIGGIDVGVKSPLVCAINNAFSRYSISDNDLFHFNKKMFARRRILLRKTRHKRAGHGVKNKLKPITILTEKSGRFRKKLIERWACEIADFFVKNKVGTVQMENLESMKRKEDSYFNIRLRGFWPYAEMQNKIEFKLKQYGIKVRKVAPNNTSKTCSKCGHLNNYFSFEYRKKNKFPHFKCEKCNFKENADYNAALNISNPKLKSTKEEP

SEQ ID NO: 1137 - protein, 726 aa, synthetic construct
SEVEFSHEYWMRHALTLAKRARDGREVPVGAVLVLNNRVIGEGWNRAISLHDPTAHAEIMALRQGGLVMQNYRLIDATLYVTFEPCVMCAGAMVHSRIGRVVFGVRNSKRGAAGSLMNVLDYPGMGHRVEITEGILADECAALLCDFYRMPRQVFNARKKAQSSINPGGSSGGSSGSETPGTSESATPESSGGSSGGSAKNTITKTLKLRIVRPYNSAEVEKIVADEKDNREKIALEKNKDKVKEACSKHLKVAAYCTTQVERNACLFCKARKLDDKFYQKLRGQFPDAVFWQEIGEIFRQLQRQAAEIYNQSLIELYYEIFIKGKGFANASSVEHYLSDVCYARAAELFKNAAIASGLRGKVKSNFRLKELKNMRSGLPTTKSDNFPIPLVKQKGGQYTGFEISSHNDDFIIKIPFGRWQAKKEIDKYRPWEKFDFEQVRKSPKPISLLLSTQRRKRNKGWSKDEGTEAEIRKVMNGDYQTSYIEVKRGSKTGEKSAWMLNLSIDVPKIDKGVDPCIIGGIDVGVKSPLVCAINNAFSRYSISDNDLFHFNKKMFARRRILLKENGHKRAGHGAKNKLKPLTVLTEKSKRFRKKLIERWACEIADFFIKNRVGTVQMENLESMKRKEDSYFNIRLRGFWPYAEMQNKIEFKLKQYGIVVRKVAPNNTSKTCSKCGHLNNYFNFEYRKKNKFPHFKCEKCNFKENADYNAALNISNPKLKSTKEEP

SEQ ID NO: 1138 - protein, 726 aa, synthetic construct
SEVEFSHEYWMRHALTLARRARDGREVPVGAVLVLNNRVIGEGWNRAIGLHDPTAHAEIMALRQGGLVMQNYRLVDATLYVTFEPCVMCAGAMIHSRIGRVVFGVRNSKRGAAGSLTNVLNYPGMSHRVKITEGILADECAALLCDFYRMPRQVFNAQKKAQSNINPGGSSGSSRGSETPGTSESAAPGSSGGNSGGSAKNTITKTLKLRIVRPYNSAEVEKIVADEKNNREKIALEKNKGKVKEACSKHLKVATYCTTQVERNACLFCKARKLDDKFYQKLRGQFPDAVFWQELGGIFRQLQKQAAEIYNQSLIELYYEIFIKGKGIANASSVEHYLSDVCYTRAAELFKNAAIASGLRNKIKSNFRLKELRNMKSGLPTTKSDNFPIPLVRQKGGQYTGFEISNHNSDFIIKIPFGRWQAKKEIDKYRPWEKFDFEQVRKSPKPISLLLSTQRRKRNRGWSKDESTEAEIKKVMNGDYQTSYIEVKRGSKVGEKSAWMLNLSIDVPKIDKGVDPSIIGGIDVGVKSPLVCAINNAFSRYSISDNDLYRFNKKMFARRRILLKKSKHKRAGHGAKNKLKPITILTEKSGRFRKKLIERWACEIADFFVKNKVGTVQMENLEGMKRKEDSYFNIRLRGFWPYAEMQNKIEFKLKQYGIEIRKVAPNNTSKTCSKCGHLNNYFNFEYRKKNKFPHFKCEKCNFKENADYNAALNISNPMLKSTKEET

SEQ ID NO: 1139 - protein, 726 aa, synthetic construct
SEVEFSHEYWMRHALTLAKRARDEHEVPVGAILVLNNRVIGVGWNRAIGLHDPTAHAEIMALRQGGLVTQNYRLIDATLYVTFEPCVMCAGAMIHSRIGRVVFGVRNSKHGAAGSLVNVLNYPGMNHRVEITEGILADECAALLCDFYRMPRQVFNARKKAQSSINSGGSSGGSSGSETPGTSESATPKSSGGSSGGSAKNTITKALKLRIVRPYNSAEVEKIVADEKNNRERIALEKNKDKVKEACSKHLKVAAYCTTQVERNACLFCKARKLDDKFYQKLRGQFPDAVFWQEIGEIFRQLQKQAAEIYNQSLIELYYEIFIKGKGFANASSVEHYLSDVCYTRAAELFKNAAIASGLRGKVKSNFRLKELKNMKSGLPTTKSDNFPIPLVKQKGGQYAGFEISSHNDDFVIKIPFGRWQVKKEIDKYRPWEKFDFEQVRKSPKPISLLLSTQRRKRNKGWSKDEGTEAEIRKVMNGDYQTSYIEVKRGSKIGEKSAWMLNLSIDVPKIDKGVNPSIIGGIDVGVKSPLVCAINNAFSRYSISDNDLFHFNKKMFARRRILLKKNRHKRAGHGAKNKLKPISILTEKSKRFRKKLIERWACEIADFFIKNKVGTVQMENLESMKRKEDGYFNIRLRGFWPYAEMQSRIEFKLKQYGIEIRKVAPNNTSKTCSKCGHLNNYFNFEYRKKNKFPHFKCEKCNFKENADYNAALNISNPMLKSTKEEP

SEQ ID NO: 1140 - protein, 726 aa, synthetic construct
SEVEFSHEYWMRHALTLAKRARDEREVPVGAVLVLNNRVIGVGWNRAIGLHDPTAHAEIMALRQGGLVMQNYRLIDATLYVTFEPCVMCAGAMIHSRIGRVVFGVRNSKHGAAGSLVNVLNYPGMNHRVEITEGILADECAALLCDFYRMPRQVFNARKKAQSSINSGGSSGGSSGSETPGTSESATPKSSGGSSGGSAKNTITKALKLRIVRPYNSAEVEKIVADEKNNREKIALEKNEDKVKEACSEHLKVAAYCTTQVERSACLFCKARKLDDKFYQKLRGQFPDAVFWQEIGEIFRQLQKQAAEIYNQSLIELYYEIFIKGKGFANASSVEHYLSDVCYTRAAELFKNAAIASGLRGKVKSNFRLKELKNMKSGLPTTKSDNFPIPLVKQKGGQYTGFEISSHNDDFIIKIPFGGWQVKKEIDKYRPWEKFDFEQVRKSPKPISLLLSTQRRKRNKGWSKDEGTEAEIRKVMNGDYQTSYIEVKRGGKIGEKSAWMLSLSIDVPKVDKGVDPSIIGGIDVGVKSPLVCAINNAFSRYSISDNELFHFNKKMFARRRILLKKSRHRRAGHGAKNKLKPITILTEKSVRFRKKLIERWACEIADFFIKNKVGTVQMENLESMKRKEDSYFNIRLRGFWPYAEMQNKIEFKLKQYGVEIRRVAPNNTSRTCSKCGHLNNYFNFEYRRKNKFPHFKCEKCNFKEDADYNAALNISNPKLKSTREEP

SEQ ID NO: 1141 - protein, 726 aa, synthetic construct
GEVEFSHEYWMHHALTLAKRARDEREVPVGAVLVLNNRVIGEGWNRAIGLHDPTAHAEIMALRQGGLVMRNYRLVDATLYVTFEPCVMCAGAMIHSRIGRVVFGVRNNKHGAAGSLVNVLNYPGMNHRVEITEGILVDECAALLCDFYRMPRQVFNAQKKARSNINSGGSSGGSSGSGTLGTSESATPESSGGSSGGSAKNTITKTLKLRIVRPYNSAEVEKIVADEKNNREKIALEKNKDKVKEACSKHLEVASYCTTQVERNACPFCKARRLDDEFYQKLRGQFPDAVFWQEIGEIFRQLQKQAAEIYNQSLIELYYEIFIKGKGFANASSVEHYLSDVCYTRAAELFKNAAIASGLRGKVKSNFRLKELKSMKSGLPTTKSDNFPIPLVKQKGGQYTGFEISCHNDDFIIKIPFGRWQVKEEIDKYRPWEKFDFEQVRKNPKPISLLLSTQRRKRNKGWSKDEGTEAEIRKVMNGDYQTSYIEVKRGSKIGEKSAWMLNLSIDVPKIDKGVDPSIIGGIDVGVKSPLVCAINNAFSRYSISDNDLFRFNKKVFARRRILLKKNRHKRAGHGTKNKLKPIAILAEKSGRFRKKLIERWACEIANFFIKNKVGTVQMENLEGMKRKEDSYFNIRLRGFWPYAEMQNKIEFKLKQYGIKIRKVAPNNTSKTCSKCGHLNNYFSFEYRKKNKFPHFKCEKCNFREDADYNAALNISNPKLKSTKEDP

SEQ ID NO: 1142 - protein, 726 aa, synthetic construct
SEVEFSHEYWMRHALSLAKRARDEREVPVGAVLVLNNRIIGEGWNRAIGLHDPTAHAEIMALRQGGLVMQNYRLTDATLYVTFEPCVMCAGAMVHSRIGRVVFGVRNSKRGAAGSLMNVLNYPGVNHCVEITEGILVDECAALLCDFYRMPRQVLNAQKKAQSSISSGGSSGGCSGSEMPGASESVTPKSSGGSSAGSTKNAITKTLKLRIVRPYNSAEVEKIVADEKNSREKIALEKNKDKVKEACSEHLKVAAYCTTQVERNACLFCKARKLDDRFYQKLRGQFPDAVFWQETGEIFRQLQRQAAEIYNQSLIELYYEIFIKGKGFANASSVEHYLSDVCYTRAAELFKNAAIASGLRGKVKSNFRLKELKNMKSGLPTTKSDNFPIPLVKQKGGQYTGFEISSHNDDFIIKIPFGRWQMKKEIDRYRPWEKFDFEQVRKSPKPISLLLSTQRRKRNKGWSKDEGTEAEIRKVMNGDYQTSYIEVKRGSKIGEKSAWMLSLSIDVPKIDKGVDPSIIGGIDVGVKSPLVCAINNAFCRYSISDNDLFHFNKKMFARRRILLKKSRHKRAGHGAKNKLKPISILTEKSKRFRKKLIERWACEIADFFIKNKVGTVQMENLESMKRKEDSYFNIRLRGFWPYAEMQNKIEFKLKQYGIEVRKVTPNNTSKTCSKCGHLNNYFNFEYRKKNKFPHFKCEKCNFKENADYNAALNISNPKLKSTKEEP

SEQ ID NO: 1143 - protein, 726 aa, synthetic construct
SEVEFSHEYWMRHALTLAKRARDEREVPVGAVLVLNNRVIGEGWNRAIGLHDPTAHAEIMALRQGGLVMQNYRLIDATLYVTFEPCVMCAGAMIHSRIGRVVFGVRNSKRGAAGSLMNVLNYPGMDHCVEITEGILVNECAALLCDFYRMPRQVLNAQKKAQSSISSGGSSGGSSCSETPGASESVTPKSSGGGSAGPTKNTITKALKLRIVRPYNSAEVEKIVADEKNNREKIALEKNKDKVKEACSKHLKVAAYCTTQVERNACLFCKARKLDDRFYQKLRGQFPDAVFWQEIGEIFRQLQKQAAEIYNQSLIELYYEIFIKGKGTANASRVEHYLSDVCYTRAAELFKNAAIASGLRGKIKSNFRLKELKNMKSGLPTTKSDNFPIPLVKQKGGQYTGFEISSHNDDFIIKIPFGRWQVKKEIDKYRPWEKFDFEQVRKSPKPISLLLSTQRRKRNKGWSKDEGTEAEIRKVMNGDYQTSYIEVKRGSKTGEKSAWMLNLSIDVPKIDKGVDPSIIGGIDVGVKSPLVCAINNAFGRYSISDNDLFRFNKKMFARRRILLKKNRHKRAGHGAKNKLKPISILTGKSERFRKKLIERWACEIADFFIKNKVGTVQMENLESMKRKEDSYFNIRLRGFWPYAEMQNKIEFKLKQYGIEIRKVAPNNTSKTCSKCGHLNNYFNFEYRKKNKFPHFKCEKCNFKENADYNAALNISNPKLKSTKEKP

SEQ ID NO: 1144 - protein, 726 aa, synthetic construct
GEVEFSHEYWMRRALTLAKRARDEREVPVGAILVLNNRVIGEGWNRAVGLHDPTAHAEIMALRQGGLVMQNYRLIDATLYVTFEPCVMCAGAMVHSRIGRVVFGVRNSKRGAAGSLMNVLDCPGMGHRVEITEGILADECAALLCDFYCMPRQVFNAQKRAQSSINSGGSSGGSSGSEAPGTSESATPESSGGGSSGSAKNTITKTLQLRIVRPYNSAEVEKIVADEKNNREKIALEKNKDKVKEACGKHLKMASYCTTQVERNACLFCKARKLDDKFYQKLRGQFPDAVFWQELGGIFRQLQKQAAEIYNQSLIELYYEIFIKGKGITNASRVEHYLSDVCYTRAAELFKNAAIASGLRSKVRSNFRLKELKNMKSGLPTTKSDNFPIPLVKQKGGQYTGFEISSHNSDFIIKIPFGRWQVKEEIDKYRPWEKFDFEQVRKSPKPISLLLSTQRRKRNKGWSKDEGTEAEIKKVMNGDYQTSYIEVKRGSKTGEKSAWMLNLSIDVPKIDKGVDPCIIGGIDVGVKSPLVCAINNAFSRYGISDNDLFHFNKKMFARRRILLKKNGHKRAGHGAKNKLKPITIMTEKSKRFRKKLIERWACEIADFFIKNKVGTVQMENLESMKRKEDSYFNIRLRGFWPYAEMQNKIEFKLKQYGIVVRKVAPNNTSKTCSKCGHLNNYFNFEYRKKNKFPHFKCEKCNFKEDADYNAALNISNPKLKSTKGEP

SEQ ID NO: 1145 - protein, 726 aa, synthetic construct
SEDEFSHEYWMRHALTLAKRARDGREVPVGAVLVLNNRVIGEGWNRAIGLHDPTAHAEIMALRQGGLVMQNYRLIDATLYVTFEPCVMCAGAMIHSRIGRVVFGVRNNKHGAAGSLVNVLNYPGMNHRVEITEGILANECAALLCDFYRMPRQVFNARKKAQSSINPGGSSGGRGGSETPGTSESATPESSGGSSGGSAKNTITKALKLRIVRPYNSAEVEKIVADEKNNREKIALEKYKDKVKEACSKHLKVASYCTTQVERNACLFCKARKLDDKFYQKLRGQFPDAVFWQEIGEIFRQLQKQAAEIYNQSLIELYYEIFIKGKGFANASSVEHYLSDVCYTRAAELFKNAAIASGLRGKVKSNFRLKELKNMKSGLPTTKSDNFPIPLVKQKGGQYTGFEISSHNDDFIIKIPFGRWQVKEEIDKYRPWEKFDFEQVRKSPKPISLLLSTQRRKRNKGWSKDEGTEAEIRKVMNGDYQTSYIEVKRGSKIGEKSAWMLSLSIDVPKIDKGVDPSIIGGIDVGVKSPLVCAINNALSRYSISDNDLFHFNKKMFARRRILLRKNRHKRAGHGARNKLKPITVLTEKSERFRKKLIERWACEIANFFIKNKVGTVQMENLESMKRREDSYFNIRLRGFWPYAEMQSKIEFKLKQYGIKIRKVAPNNTSKTCSKCGHLNNYFNFEFRKKNKFPHFKCEKCNFKEDADYNAALNISNPKLKGTKEEP

SEQ ID NO: 1146 - protein, 726 aa, synthetic construct
SEVEFSHEYWMRHALTLAKRARDEREVPVGAVLVLNNRVIGEGWNRAIGLHDPTAHAEIMALRQGGLVMQNYRLVDATLYVTFEPCVLCAGAMVHSRIGRVVFGVRNSKRGAAGSLMNVLDYPGMNHRVEITEGILADECAALLCDFYRMPRQVFNAQKKARPNINSGGSSGGRSGSETPGTSESATPESSGGSSAGSTKDTITKTLKLRIVRPYNSAEVEKVVADEKNNREKIAMEKNKDKVKEACSKHLKVASYCTTQVERNACLFCKARKLDDKFYQKLRGQFPDAVFWQELGGIFRQLQKQAAEIYNQSLIELYYEIFIKGKGITNASRVEHYLSDVCYTRAAELFKNAAIASGLRSKVRSNFRLKELKNMKSGLPTTKSDNFPIPLVKQKGGQYTGFEISSHNSDFIIKIPFGRWQEKEEIDKYRPWEKFDFEQVRRSPKPISLLLSTQRRKKNKGWSKDEGTEAEIRRVMNGDYQTSYIEVKRGSKIGEKSAWMLNLSIDVPKIDKGVDPSIIGGIDVGVKSPLVCAINNALSRYSISDNDLFHFNKKMFARRRILLRKNRHKRAGHGAKNKLKPITIMTEKSKRFRKKLIERWACEIADFFIKNKVGTVQMENLESMKRREDSYFNIRLRGFWPYAEMQNKIEFKLKQYGIVVRKVAPNNTSKTCSKCGHLNNYFNFEYRKKNKFPRFKCEKCNFKENADYNAALNISNPKLKSPKEEP

SEQ ID NO: 1147 - protein, 726 aa, synthetic construct
SEIEFSHEYWMRHALTLARRARDEREVPVGAILVLNNRVIGEGWNRAIGLHDPTAHAEIMALRQGGLVMQNYRLTDATLYVTFEPCVMCAGAMIHSRIGRVVFGVRNSKRGAAGSLMNVLNYPGMNHCVEITEGILVDECAALLCDFYRMPRQVLNARKKAQSSINSGGSSGGSSGSETPSTSESATPESSGGSSGGSAKNTITKTLQLRIVRPYNSAEVEKIVTDEKNNREKIALEKNKDKVKEACSKHLKMASYCTTQVERNACLFCKARKLDDKFYQKLRGQFPDAVFWQELGGIFRQLQKQAAEIYNQSLIELYYEIFIKGKGITNASRVEHYLSDVCYTRAAELFKNAAIASGLRSKVRSNFRLKELKNMKSGLPTTKSDNFPIPLVKQKGGQYTGFEISSHSDDFIIKIPFGRWQVKEEIDKYRPWEKFDFEQVRKSPKPISLLLSTQRRKRNRGWSKDESTEAEIKKVMYGDYQTSYIEVKRGSKIGEKSAWMLNLSIDVPKIDKGVDPSIIGGIDVGVKSPLVCAINNAFSRYSISDNDLFHFNKKVFARRRILLKKNRHRRAGHGAKNKLKPITILTEKSKRFRKKLIERWACEIADFFIKNKVGTVQMENLESMKRKEDSYFNIRLRGFWPYAEMQNKIEFKLKQYGIKIRKVAPNNTSRTCSECGHLNNYFSFEYRKKNKFPHFKCEKCNFKEDADYNAALNISNPKLKGTKEEL

SEQ ID NO: 1148 - protein, 726 aa, synthetic construct
SEVEFSHEYWMRHALTLAKRARDEREVPVGAILVLNNRVIGEGWNRAIGLHDPTAHAEIMALRQGGLVMQNYRLIDATLYVTFEPCVMCAGAMIHSRIGRVVFGVRNSKHGAAGSLVNVLNYPGMNHRVEITEGILADECAALLCDFYRMPRQVFGARRKAQSSINPGGSSGGSSGSETLGTSESATPESSGGGSSGSAKNTITKTLQLRIVRPYNSAEVEKIVADEKNNREKIALEKNKDKVKEACSRHLKVASYCTTQVERNACPFCKARKLDDKFYQKLRGQFPDAVFWQELGEILRQLQKQAAEIYNQSLIELYYEIFIKGKGFANASSVEHYLSDVCYTRAAELFKNAAIASGLRGKIKSNFRLKELKNMKSGLPTTKSDNFPIPLVKQKGGQYTGFEISNHNSDFIIKIPFGRWQAKKEIDKYRPWEKFDFEQVRKSPKPISLLLSTQRRKRNRGWSRDEGTEAEIKKVMNGDYQTSYIEVKRGSKIGEKSAWMLNLSIDVPKIDKGVDPSIIGGIDVGVKSPLVCAINNAFSRYSISDNDLFHFNKKMFARRRILLRKSKHKRAGHGAKNKLKPITILTEKSRRFRKKLIERWACEIADFFIKNKVGTVQMENLESMKRKEDSYFNIRLRGFWPYAEMQNKIEFKLKQYGIEIRKVAPNNTSKTCSKCGHLNNYFNFEYRKMNKFPHFKCEKCNFKENADYNAALNISSPKLKSTKEGP

SEQ ID NO: 1149 - protein, 726 aa, synthetic construct
SEDEFSHEYWMRHALTLAKRARDEREVPVGAILVLNNRVIGEGWNRAIGLHDPTAHAEIMALRQGGLVMQNHRLVDATLYVTFEPCVMCAGAMIHSRIGRVVFGVRNSKRGAAGSLTNVLNYPGMNHCVEITEGILVDECAALLCDFYRMPRQVLNAQKKAQSSISSGGSSGGSSGSETPGTSESATPESSGGSSGGSAKNTITKTLKLKIVRPYNSSEVEKIVADEKNNREKIALEKNKDKVKEACSKHLKVAAYCTTQVERNACLFCKARRLDDKFYQKLRGQFPDAVFWQEIGEIFRQLQKQAAEIYNQSLIELYYEIFIKGRGFANASSVEHYLSDVCYTRAAEQFKNAAIASGLRGKVKGNFRLKELKNMKSGLPTTKSDNFPIPLVKQKGGQYTGFEISSHNDDFIIKIPFGRWQVKKEIDKYRPWEKFDFEQVRKSPKPISLLLSTQRRKRNKGWSKDEGTEAEIRKVMNGDYQTSYIEVKRGSKTGEKSAWMLSLSIDVPKIDKGVDPSIIGGIDVGVKSPLVCAINNAFSRYSISDNDLFRFNKKMFARRRILLKKNRHKRAGHGAKNKLKPISILTGKSERFRKKLIERWACEIADFFIKNKVGTVQMESLESMKRKEDSYFNIRLRGFWPYAEMQNKIEFKLKQYGIEIRKVAPNNTSKTCSKCGHLNNYFNFEYRKKNKFPHFKCEKCNFKENADYNAALNISNPKLKSTKEEP

SEQ ID NO: 1150 - protein, 726 aa, synthetic construct
SEVEFSHEYWMRHALTLAKRARDEREVPVGAILVLNNRVIGEGWNRAIGLHDPTAHAEIMALRQGGLVTQNYRLIDATLYVTFEPCVMCAGAMIHSRIGRVVFGVRNSKHGAAGSLVNVLNYPGMNHRVEITEGVLADECAALLCDFYRMPRQVFNARKKAQSNINPGGSSGGSSGSETPGTSDSATPGSSGGSSGGSAKNTITKTLKLRIVRPYNSAEVEKIVADEKNNREKTALEKNKDKVKEACSEHLKVATYCTTQVERNACLFCKARKLDDKFYQKLRGQFPDAVFWQEIGEVFRQLQKQAAEIYNQSLIELYYEIFIKGKGFANASSVEHYLSDVCYTRAAELFKNAAIASGLRNKTKSNFRLKELRSMKSGLPTTKSDNFPIPLVKQKGGQYTGFEISNHNSDFIIKIPFGRWQAKKEIDKYRPWEKFDFEQVRKSPKPISLLLSTQRRKRNKGWSKDEGTEAEIEKVMNGDYQTSYIEVKRGSKTGGKSAWMLNLSIDVPKIDKGVDPCIIGGIDVGVKSPLVCAINDAFSRYSISDNDLFHFNKKMFARRRILLKKNGHKRAGHGAKNKLKPITIMTEKSKRFRKKLIERWACEIADFFIKNKVGTVQMENLESMKRKEDSYFNIRLRGFWPYAEMQNKIEFKLKQYGIVVRKVAPNNTSKTCSKCGHLNNYFNFEYRKKNKFPHFKCEKCNFKENADYNAALNISNPQLKSTKGEP

SEQ ID NO: 1151 - protein, 726 aa, synthetic construct
SEVEFSHEYWMRHALTLAKRARDEREVPVGAVLVLNNRVIGVGWNRAIGLHDPTAHAEIMALRQGGLVMQNYRLTDATLYVTFEPCVMCAGAMVHSRIGRVVFGVRNSKRGAAGSLMNVLNYPGMSHCVEITEGILVDECAALLCDFYRMPRQVLNAQKKAQSSINSGGSSDGSSGSETPGTSESATPESSGGGSSGSARNTITKTLQLRIVRPYNSAEVEKIVADEKNNREKIALERNKGKVREACNKHLKVASYCTTQVERNACPFCKARKLDDKFYQKLRGQFPDAVFWQELGEILRQLQRQAAEIYNQSLIELYYEIFIKGRGFANASSVEHYLSDVCYTRAAELFKNAAIASGLRGKVKSNFRLKELKNMKSGLPTTKSDNFPIPLVKQKGGQYTGFEISSHNDDFIIKIPFGRWQVKKEIDKYRPWEKFDFEQVRKSPKPISLLLSTQRRKRNKGWSKDEGTEAEIRKVMNGVYQTSYIEVKRGSKIGEKSAWMLNLSIDVPKIDKGVDPSIIGGVDVGVKSPLVCAINNALSRYSISDNDLFHFNKKMFARRRILLRKNRHKRAGHGAKNKLKPITIMTEKSKRFRKKLIERWACEIADFFIKNKVGTVQMENLESMKRREDSYFNIRLRGFWPYAEMQNKIEFKLKQYGIVVRKVAPNNTSKTCSKCGHLNNYFNFEYRKKNKFPHFKCEKCNFKEDADYNAALNISNPKLKSTKGEP

SEQ ID NO: 1152 - protein, 726 aa, synthetic construct
SEVEFSHEYWMRHALTLAKRARDEREVPVGAILVLNNRVIGEGWNRAIGLHDPTAHAEIMALRQGGLVMQNYRLIDATLYVTFEPCVMCAGAMIHSRIGRVVFGVRNNKHGAAGSLVNVLDYPGMNHRVEITEGILADECAALLCDFYRMPRQVFNARKKAQSSISSGGSSGGSGGGETPGASESVTPKNSGGSSGSSAKNTITKTLKLRIVRPYNSAEVEKIVADEKNNREKIALEKNKDKVKEACSEHLKVAAYCTTQVERSACLFCKARKLDDKFYQKLRGQFPDAVFWQEIGEIFRQLQKQAAEIYNQSLVELYYEIFIKGKGIANASSVEHYLSDVCYTRAAELFKNAAIASGLRNKIKSNFRLKELRNMKSGLPTTKSDNFPIPLVRQKGGQYTGFEISNHNGDFIIKIPFGRWQVKKEIRKHRPWEKFDFEQVRKSPKPISLLLSTQRRKRNKGWSKDEGTEAEIRKVMNGDYQTSYIEVKRGSRIGEKSAWMLSLSIDVPKIDRGVDPSIIGGIDVGVKSPLVCAINNGLSRYSISDNDLFHFNKKMFARRRILLKKNRHRRAGHGARNKLKPITVLTEKSKRFRKKLIERWACEIANFFVKNKVGTVQMENLESMKRKEDSYFNIRLRGLWPYAEMQNKIEFKLKQYGIEVRKVAPNNTSKTCSKCGHLNNYFNFEYRKKNKFPPFKCEKCNFKENADYNAALNISNPKLKGTKEEP

SEQ ID NO: 1153 - protein, 726 aa, synthetic construct
SEVEFSHEYWMRHALSLAKRARDEREVPVGAVLVLNNRIIGEGWNRAIGQHDPTAHAEIMALRQGGLVMQNYRLTDATLYVTFEPCVMCAGAMVHSRIGRVVFGVRNSKRGAAGSLMNVLNYPGVNHCVEITEGILVDECAALLCDFYRMPRRVLNAQKKAQSSISSGGSSGGSNGSETRGASESATPKSSGGSSAGSTKNTITKTLKLRIVRPYNSAEVEKIVADEKNSREKTALEKNKDKVKEACSKHLKVAAYCTTQVERSACLFCRARKLDDKFYQKLRGQFPDAVFWQEIGEIFRQLQKQAAEVYNQSLVELYYEILIKGKGIANASSVEHYLSDVCYTRAAELFKNAAIASGLRNKIKSNFRLKELRNMKSGLPTTKSDNFPIPLVRQKGGQYTGFEISNHDGDFIIKIPFGRWQVKKEIDKYRPWEKFDFEQVRKSPKPISLLLSTQRRKRNKGWSRDEGTEAEIRKAMNGDYQTSYIEVKRGSKIGEKSAWMLSLSIDVPKIDKGVDPRIIGGIDVGVKSPLVCAINNAFSRYSISDNDLYRFNKKMFARRRILLKKSRHKRAGHGAKNKLKPISILTEKSKRFRKKLIERWACEIADFFIKNKVGTVQMENLESMKRKEDSYFNIRLRGFWPYAEMQNKIEFKLKQYGIKIRKVAPNNTSKTCSKCGHLNNYFSFEYRKKNKFPHFKCEKCNFKENADYNAALNIGNPKLMSTKEEP

SEQ ID NO: 1154 - protein, 726 aa, synthetic construct
SEVEFSHEYWMRHALTLAKRARDEREVPVGAILVLNNRVIGEGWNRAIGLHDPTAHAEIMALRQGGLVMQNYRLIDATLYVTFEPCVMCAGAMIHSRIGRVVFGVRNSKHGAAGSLVNVLNYPGMNHRVEITEGILADECAALLCDFYRMPRQVFSARRKAQSSINPGGSSGGSSGSETPGTSESPTPESPGGSSGGSAKNTITKTLKLRIVRPYNSAEVEKIVADEKNNREKIALEKNKGKVKEACSKHLEVAAYCTTQVERNACLFCKARKLDDKFYQKLRGQFPDAVFWQELGEIFRQLQKQAAEIYNQSLIELYYEIFIKGKGFANASSVEHYLSDVCYTRAAELFKNAAIASGLRGKVKSNFRLKELKNMKSGLPTTKSDNFPIPLVKQKGGQYTGFEISSHNDDFIIKIPFGRWQVRKEIDKYRPWEKFNFEQVRKSPKPISLLLSTQRRKRNKGWSKDEGTEAEIRRVMNGDYQTSYIEVKRGSKIGEKSAWMLNLSIDVPKIDKGVDPSIIGGIDVGVKSPLVCAINNAFSRYSISDNDLFHFNKKMFARRRILLKKNRHRRAGHGAKNKLKPITILTEKSVRFRKKLIERWACEIADFFIKNKVGTVQMENLESMKRREDSYFNIRLRGFWPYAEMQNKIEFKLKQYGIEIRKVAPNNTSKTCSKCGHLNNYFNFEYRKMNKFPHFKCEKCNFKENADYNAALNISNPKLKSTKEEP

SEQ ID NO: 1155 - protein, 726 aa, synthetic construct
SEVEFSHEYWMRHALTLAKRARDEREVPVGAVLVLNNRVIGEGWNRAIGLHDPTAHAEIMALRQGGLVMQNYRLVDATLYVTFEPCVLCAGAMVHSRIGRVVFGVRNSKRGAAGSLMNVLNYPGMNHRVEITEGILADECAALLCDFYRMPRQVFNARKKARSNINSSGSSGGSSGSETPGTSESATPESSGGSSGGSAKNTITKTLKLRIVRPYNSAEVEKIVADEKNNREKIALEKNKDKVKEACSEHLKVAAYCTTQVGRNACLFCKARRLDDRFYQKLRGQFPDAVFWQEIGEIFRQLQKQAAEIYNQSLIELYYEIFIKGKGFANASSVEHYLSDVCYTRAAELFKNAAIASGLRGKVKSNFRLKELKNMRSGLPTTKSDNFPIPLVKQKGGQYTGFEISSHNDNFIIKIPFGRWQVKKEIDKYRPWEKFDFEQVRKSPKPISLLLSTQRRKRNKGWSKDEGTEAEIRKVMNGDYQTSYIEVKRGSKTGEKSAWMLNLSIDVPKIDKGVDPSIIGGIDVGVKSPLVCAINNAFSRYSISDNDLFRFNKKMFARRRILLGKNRHKRAGHGVKNKLKPITILTEKSGRFRKKLIERWACEIADFFIKNKVGTVQMENLESMKRKEDSYFNIRLRGFWPYAEMQNKIELKLKQYGIKIRKVAPNNTSKTCSRCGHLNDYFNFEYRKKNKFPHFKCEKCNLKEDADYNAALNISNPKLKSTKEEP

SEQ ID NO: 1156 - protein, 726 aa, synthetic construct
SEVEFSHEYWMRHALTLAKRARDEREVPVGAILVLNNRVIGEGWNRTIGLHDPTAHAEIMALRQGGLVMQNCRLVDATLYVTFEPCVMCAGAMIHSRIGRVVFGVRNSKRGAAGSLMNVLNYPGTNHRVEITEGILADECAALLCDFYRMPRRVFNAQKKARSNINSGGSSGGSSGSETPSTSESATPESSGGSSGGSAKNTITKTLTLRIVRPYNSAEVEKIVADEKNNREKIALEKNKDKVKEACSEHLKVASYCTTQVERNACPFCKARKLDDKFYQKLRGQFPDAMFWQELGEILRQLQKQAAEIYNQSLIELYYEIFIKGRGFANASSVEHYLSDVCYTRAAELFKNAAIASGLRGKVKSNFRLKELKNMKSGLPTTKSDNFPIPLVKQKGGQYTGFEINSHNDDFIIKIPFGRWQVKKEIDKYRPWEKFDFEQVRKSPKPISLLLSTQRRRRNKGWSRDEGTEAEIKKVMNGDYQTSYIEVKRGSKTGEKSAWMLNLSIDVPKIDKGVDPSIIGGIDVGVKSPLVCAINNAFSRYSISDNDLFRYNKKMFARRRILLKKNRHKRAGHGARNKLKPISILTEKSKRFRKKLIERWACEIADFFIKNKVGTVQIENLESMKRREDSYFNIRLRGFWPYAEMQNKIEFKLKQYGIEIRKVAPNNTSKTCSKCGHLNSYFNFEYRKKNKFPHFKCEKCNFRENADYNAALNISNPKLRSTKEEP

SEQ ID NO: 1157 - protein, 726 aa, synthetic construct
SEVEFSHEYWMRHALTLAKRARDEREVPVGAVLVLNNRVIGVGWNRAIGLHDPTAHAEIMALRQGGLVMQNYRLIDATLYVTFEPCIMCAGAMIHSRIGRVVFGVRNSKRGAAGSLMNVLNYPGMNHRVEITEGVLADECAALLCDFYRMPRQVLNAQKKAQSSINSGGSSGGGSGGETPGTSESATPESSGGSSGGSAKNTITKTLKLRIVRPYNSAEVEKIVADEKDNRERIALEKNKDKVKEACSKHLKVAAYCTTQVERNACLFCRARKLDDKFYQKLRGQFPDAVFWQEIGEVFRQLQKQAAEIYNQSLIELYYEIFIKGKGITNASRVEHYLSDVCYTRAAELFKNAAIASGLRSKVRSNFRLKELKNMKSGLPTTKSDNFPIPLVKQKGGQYAGFEISSHNGDFIIKIPFGRWQVKKEIDKYRPWEKFDFEQVRKSPKPISLLLSTQRRKRSKGWSKDEGTEAEIRKVMNGDYQTSYIEVKRGSKTGEKSAWMLNLSIDVPKIDKGVDPSIIGGIDVGVKSPLVCAINNAFSRYSISDNDLFRFNKKMFARRRILLKKNRHKRAGHGAKNKLKPISILTGKSKRFRKKLIERWACEIADFFIKNKVGTVQMENLESMKRKEDSYFNIRLRGFWPYAEMQNKIEFKLKQYGIKIRKVAPNNTSRTCSKCGHLNNYFSFEYRKKNKFPHFKCEKCNFKEDADYNAALNISNPKLKGTKEEL

SEQ ID NO: 1158 - protein, 726 aa, synthetic construct
SEVEFSHEYWMRHALTLAKRARDEREVPVGAVLVLNNRVIGEGWNRTTGLHDPTAHAEIMALRQGGLVMRNYRLTDATLYVTFEPCVMCAGAMIHSRIGRVVFGVRNSKRGAAGSLMNVLNYPGMSHCVEITEGILVDECAALLCDFYRMPRQVLNAQKKAQSSISSGGSSGGSGGGETPGASGSVTPKSSGGSSGGSAKNTITKALKLRIVRPYNSAEVEKIVADEKNNREKIALEKNKDKVKEACSKHLKVAAYCTTQVERNACPFCKARRLDDKFYQKLRGQFPDAVFWQEIGEIFRQLQKQAAEIYNQSLVELYYEIFIKGKGIANTSSVEHYLSDVCYTRAAELFKNAAIASGLRNKIKSNFRLKELRNMKSGLPTTKSDNFPIPLVRQKGGQYTGFEISNHNGDFIIKIPFGRWQVKKEICKHRPWEKFDFEQVRKSPKPISLLLSTQRRKRNKGWGKDEGTEAEVRKVMNGDYQTSYIEVKRGSKIGEKSAWMLNLSIDVPKIDKGVDPSIIGGIDVGVKSPLVCAINNALSRYSISDNDLFHFNKKMFARRRILLRKNRHKRAGHGARNKLKPITVLTEKSERFRKKLIERWACEIANFFIKNKVGTVQMENLESMKRREDSYFNIRLRGFWPYAEMQNKIEFKLKQYGIKVRKVAPNNTSKTCSKCGHLNNYFSFEYRKKNKFPHFKCEKCNFKENADYNAALNISNPKLKSTKEEP

SEQ ID NO: 1159 - protein, 726 aa, synthetic construct
SEVEFSHEYWMRHALTLAKRARDEREVPVGAILVLNNRVIGEGWNRAIGLHDPTAHAEIMALRQGGLVMQNYRLIDATLYVTFEPCVMCAGAMIHSRIGRVVFGVRNSKHGAAGSLVNVLNYPGMNHRVEITEGILADECAALLCDFYRMPRQVFNARKKAQSSINPSGSSGGSSGSVTPGTSESATPESSGGGFGGSAKNTITKTLQLRIVRPYNSAEVEKIVADEKNNREKIALEKNKDKVKEACSKHLKVASYCTTQVERNACLFCKARKLDDKFYQKLRGQFPDAVFWQELGEIFRQLQKQAAEIYNQSLIELYYEIFIKGKGLANASSVEHYLSDVCYTRAAELFKNAAIASGLRGKVKSNFKLKELKSMKSGLPSTKSDNFPIPLVRQKGGQYTGFEISSHNDDFIIKIPFGRWQAKKEIDRYRPWEKFDFEQVRKSPKPISLLLSTQRRKRNKGWSKDEGTEAEIRKVMNGDYQTSYIEVKRGSKTGEKSAWMLNLSIDVPKIDKGVDPSIIGGIDVGVRSPLVCAIDNAFSRYSISDNDLFHFNKKMFARRRILLKKNRHKRAGHGAKNKLKPISILTEKSKRFRKKLIERWACEIADFFIKNKVGTVQMENLESMKRKEDSYFNIRLRGFWPYAEMQNKIEFKLKQYGIEIRKVAPNNTSKTCSKCGHLNNYFNFEYRKKNKFPHFKCERCSFKENADYNAALNISNPKLKSTKEEP

SEQ ID NO: 1160 - protein, 726 aa, synthetic construct
GEVEFSHEYWMRHALTLAKRARDEREVPVGAVLVLNNRVIGEGWNRAIGLHDPTAHAEIMALRQGGLVMQNYRLSDATLYVTFEPCVMCAGAMIHSRIDRVVFGVRNSKRGAAGSLMNVLNYPGMNHCVEITEGILVDECAALLCDFYRMPRQVLSAQKKAQSSISSGGSSGGSSGSETPGASGSVTPKSSVGSSAGSTKNTITKTLKLRIVRPYNSAEVEKIVADEKNNREKIALEKNKDKVKEACSKHLKVAAYCTTQVERNACLFCKARKLDDKFYQKLRGQFPDAVFWQEISEIFRQLQKQAAEIYNQSLIELYYEIFIKGKGFANASSVEHYLSDVCYTRAAELFKNAAIASGLRGKVKSNFRLKELKNMKSGLPTTKSDNFPIPLVRQKGGQYTGFEVSSHNDDFIIKIPFGRWQVKKEIDKYRPWEKFDFEQVRKGPKPISLLLSTQRRKRNKGWSKDEGTEAEIRKVMNGNYQTSYIEVKRGSKIGEKNAWMLSLSIDVPKIDKGVDPSIIGGIDVGVKSPLVCAINNALSRYSISDNDLFHFNKKMFARRRILLKKNRHKRAGHGARNKLRPITVLTEKSERFRKKLIERWACEIANFFIKNKVGTVQMENLESMKRKEDSYFNIRLRGFWPYAEMQNKIEFKLKQYGIEIRKVAPNNTSKTCSKCGHLNNYFDFEYRKKNKFPHFKCEKCNFKENADYNAALNISNPKLKSTKGEP

SEQ ID NO: 1161 - protein, 726 aa, synthetic construct
SEVEFSHEYWMRHALTLAKRARDEREVPVGAVLVLNNRVIGEGWNRTTGLHDPTAHAEIMALRQGGLVMQNYRLTGATLYVTFEPCVMCAGAMIHSRIGRVVFGVRNSKHGAAGSLVNVLNYPGMNHRVEITEGILADECAALLCDFYRMPRQVFNARKKAQSSINSGGSSGGSSGSETPGTSESATPKSSGGSSGGSAKNTITKALKLRIVRPYNSAEVEKIVADEKNNRERIALEKNKDKVKEACSKHLKVAAYCTTQVERNACLFCKARKLDDKFYQKLRGQFPDAVFWQEIGEIFRQLQKQAAEVYNQSLIELYYEIFIKGKGFANASSVEHYLSDVCYTRAAELFKNAAIASGLRGKVKSNFRLKELKNMRSGLPTTKSDNFPIPLVKQKGGQYAGFEISSHNDDFIIKIPFGRWQVKKEIDKYRPWEKFDFEQVRKSPKPISLLLSTRRRKRNKGWSKDEGTEAEIRKVMNGDYQTSYIEVKRGSKIGEKSAWMLNLSIDVPKIDKGVDPSIIGGIDVGVKSPLVCAINNAFGRYSISDNDLFHFNKKMFARRRILLKRNRHKRAGHGAKNKLKPITILTEKSKRFRRKLIERWACEIADFFIKNKVGTVQMENLESMKRKEDSYFNIRLRGFWPYAEMQDKIEFKLKQYGIEIRKVAPNNTSKTCSKCGHLNNYFNFEYRRKNKFPHFKCEKCNFKENADYNAALNISNPKLKSTKEEP

SEQ ID NO: 1162 - protein, 726 aa, synthetic construct
SEVEFSHEYWMRHALTLAKRARDEREVPVGAVLVLNNRVIGGGWNRAIGLHDPTAHAEIMALRQGGLVMQNCRLVDATLYVTFEPCVMCAGAMIHSRIGRVVFGVRNSKRGAAGSLMNVLNYPGMNHRVEITEGILAGECAALLCDFYRMPRQVFNAQKKAQSTINSGGSSGGSSSSETPGISGSATPEGSGGSSGGSAKNTITKTLKLRIVRPYNSAEVEKIVADEKNNREKIALEKNKDKVKEACSKHLKVASYCTTQVERNACLFCKARKLDDKFYQKLRGQFPDAVFWQELGEIFRQLQKQAAEIYNQSLIELYYEIFIKGKGFANASSVEHYLSDVCYTRAAELFKNAAIASGLRGKVKSNFRLKELKNMKSGLPTTKSDNFPIPLVKQKGGQYTGFEISSHNDDFIIKIPFGRWQVKKEIDKYRPWEKFDFEQVRKSPKPISLLLSTQRRKKNKGWSKDEGTEAEIRRVMNGDYQTSYIEVKRGSKIGEKSAWMLNLSIDVPKIDKGVDPSIIGGIDVGVKSPLVCAINNSSSRYSICDNDLFRFNKKMFARRRILLKKNRHKRAGHGAKNKLKPITILTKKSERFRKKLIERWVCEVADFFIKNKVGTVQMENLGSMKRKEDSYFNIRLRGFWPYAEMQNKIEFKLKQYGIEIRKVAPDNTSKTCSKCGHLNNYFNFEYRKKNKFPHFKCEKCNFKEDADYNAALNISNPKLKSTKEEP

SEQ ID NO: 1163 - protein, 726 aa, synthetic construct
SEVEFSHEYWMRHALTLAKRARDEREVPVGAVLVLNNRVIGEGWNRAIGLHDPTAHAEIMALRQGGLVLQNYRLVDATLYVTFEPCIMCAGAMIHSRIGRVVFGVRNSKRGAAGSLMNVLNYPGMNHRVEITEGILADECAALLCDYYRMPRQVFNAQKKARSNINPGGSSGGSGGSETPGTSESATSESSGGSSGGSAKNTITKTLKLRIVRPYNNAEVEKIVADEKNNREKIALEKNKDKVKEACSKHLKVASYCTTQVERNACLFCKARKLDDKFYQKLRGQFPDAVFWQELGGIFRQLQKQAAEIYNQSLIELYYEIFIKGKGITNASRVEHYLSDVCYTRAAELFKNAAIASGLRSKVRSNFRLKELKNMKSGLPTTKSDNFPIPLVKQKGGQYTGFEISSHNDDLIIKIPFGRWQVKKEIDKYRPWEKFDFEQVRKSPKPISLLLSTQRRKRNRGWSKDEGTEAEIRKVMNGDYQTSYIEVKRGSKTGGKSAWMLNLSIDVPKIDKGVDPCIIGGIDVGVKSPLVCAINDAFSRYSISDNDLFHFNKKMFARRRILLKKNGHKRAGHGAKNKLKPITIMTEKSKRFRKKLIERWACEIADFFIKNKVGTVQMENLESMKRKEDSYFNIRLRGFWPYAEMQNKIEFKLKQYGIVVRKVAPNNTSKTCSKCGHLNNYFNFEYRKKNKFPYFKCEKCNFKENADYNAALNISNPKLKSTKEEL

SEQ ID NO: 1164 - protein, 726 aa, synthetic construct
SEVEFSHEYWMRHALTLAKRARDEREVPVGAILVLNNRVIGEGWNRAIGLHDPTAHAEIMALRQGGLVMQNYRLIDATLYVTFEPCVMCAGAMIHSRIGRVVFGVRNNKHGAAGSLVNVLNYPGMNHRVGITEGILADECAALLCDFYRMPRQVFNARKKAQPSINPGGSSGGSSGSETPGTSESATPESSGGSSGGSAKNTITKTLKLRIVRPYNSAEVEKIVADEKNNREKIALEKNKDKVKEACSKHLKVAAYCTTQVERNACLFCKARRLDDKFYQKLRGQFPDAVFWQEIGEIFRQLQKQAAEIYNQSLIELYYEIFIKGKGIANASSVEHYLSDVCYTRAAELFKNAAIASGLRNKVKSNFRLKELRSMKSGLPTTKSDNFPIPLVRQKGGQYTGFEISNHNSDFIIKIPFGRWQAKKEIDKYRPWEKFDFEQVRKSPKPISLLLSTQRRKRNRGWSKDESTEAEIKKVMNGDYQTSYIEVKRGSKVGEKSAWVLNLSIDVPKIGKGVDPSIIGGIDVGVKSPLVCAINNAFSRYSISDNDLYRFNKKMFARRRILLKKSKHKRAGHGAKNKLKPITILTEKSGRFRKKLIERWACEIADFFIKNKVGTVQMENLEGMKRKEDSYFNIRLRGFWPYAEMQNKIEFKLKQYGIEIRKVAPNNTSKTCSKCGHLNNYFNFEYRKKNKFPHFKCEKCNFKENADYNAALNISNPKLKSTKEEP

SEQ ID NO: 1165 - protein, 726 aa, synthetic construct
SEVEFSHEYWMRHALTLAKRARDEREVPVGAVLVLNNRVIGEGWNRAIGLHDPTAHAEIMALRQGGLAMQNYRLVDATLYVTFEPCVLCAGAMVHSRIGRVVFGVRNNKRGAAGSLMNVLNYPGMNHRVEITEGILADECAALLCDFYRMPRRVFNARKKAQSSIDPGGPSDGSSGSETPGISESATPESSGGGSSGSAKNTITKTLQLRIVRPYNSAEVEKIVADEKNNRERIALEKSKDKVKEACSKHLKVASYCTTQVERNACPFCKARKLDDKFYQKLRGQFPDAVFWQELGEILRQLQKQAAEIYNQSLIELYYEIFIKGRGFANASSVEHYLSDVCYTRAAELFKNAAIASGLRGKVKSNFRLKELKNMKSGLPTTKSDNFPIPLVKQKGGQYTGFEISSHNDDFIIKIPFGRWQVKKEIDKYRPWEKFDFEQVRKSPKPISLLLSTQRRKRNKGWSKDEGTEAEIRKVMNGDYQTSYIEVKRGSKTGEKSAWMLNLSIDVPKIDKGVDPSIIGGIDVGVKSPLVCAINNAFSRYSISDNDLFRFNKKMFARRRILLKKNRHKRAGHGAKNKLKPISILTGKGERFRKKLIERWACEIADFFIKNKVGTVQMENLESMKRKEDSYFNIRLRGFWPYAEMQNKIEFKLKQYGIEIRKVAPNNTSKTCSKCGHLNNYFNFEYRKKNKFPHFKCEKCNFKEDADYNAALNISNPKLKSTKEEP

SEQ ID NO: 1166 - protein, 726 aa, synthetic construct; identical to SEQ ID NO: 684

SEQ ID NO: 1167 - protein, 726 aa, synthetic construct
SEVEFSHEYWMRHALTLARRARDEREVPVGAILVLNNRVIGEGWNRANGLHDPTAHAEIMALRQGGLVMQNYRLIGATLYVTFEPCVMCAGAMVHSRIGRVVFGVRNSKRGAAGSLMNVLDYPGMGHRVEITEGILADECAALLCDFYRMPRQVFNAQKKARSNINSGGSSGGSSGSETPGTSESATPESSGGGSGGSAKNTITKTLQLRIVRPYNSAEVEEIVADEKNNREKIALEKNKDKVREACSKHLKVASYCTTQVERNACLFCKARKLDDKFYQKLRGQFPDAVFWQEIGEIFRQLQKQAAEIYNQSLIELYYEIFIKGRGFANAGSVEHYLSDVCYTRAAELFKNAAIASGLRGKVKSNFRLKELKNMKSGLPTTKSDNFPIPLVKQKGGQYTGFEISSHNDDFIIKIPFGRWQVKEEIDKYRPWEKFDFEQVRKNPKPISLLLSTQRRKRNKGWSKDEGTEAEIRKVMNGDYQTSYIEVKRGSKIGEKSAWMLNLSIDVPKIDKGVDPSIIGGIDVGVKSPLVCAINNAFSRYSISDNDLFRFNKKVFARRRILLKKNRHKRAGHGTKNKLKPITILTEKSGRFRKKLIERWACEIANFFIKNKVGTVQMENLESMKRKGDSYFNIRLRGFWPYAEMQNKIEFKLKQYGIKIRKVAPNNTSKTCSKCGHLNNYFSFEYRKKNKFPHFKCEKCNFKEDADYNAALNISNPKLRSTKEEP

SEQ ID NO: 1168 - protein, 726 aa, synthetic construct
SEVEFSHEYWMRHALALAKRARDGREVPVGAVLVLNNRVIGEGWNRAIGLHDPTAHAEIMALRQGGLVIQNYRLIDATLYVTFEPCAMCAGAMVHSRIGRVVFGVRNSKRGAAGSLMNVLNYPGMDHRVEITGGILADECAALLCDFYRMPRRVFNAQKKAQSSINSGGSSGGSSGSVTPGTSESATPESSGGSFGGSAKNTITKTLQLRIVRPYNSAEVEKIVADEKNSREKIALEKNKDKVKEACGKHLKVASYCTTQVERNACLFCKARKLDDKFYQKLRGQFPDAVFWQELGEIFRQLQKQAAEIYNQSLIELYYEIFIKGKGLANASSVEHYLSDVCYTRAAELFKNAAIASGLRGKVKSNFKLKELKSMKSGLPSTKSDNFPIPLVKQKGGRYTGFEISSHNDDLIIKIPFGRWQVKKEIDKYRPWEKFDFEQVRKSPKPISLLLSTQRRKRNKGWSKDEGTEAEIRKVMNGDYQTSYIEVKRGSKIGEKSAWMLNLSIDVPKIDKGVDPSIIGGIDVGVKSPLVCAINNAFSRYSISDNDLFRFNKKMFARRRILLKKNRHKRAGHGAKNKLKPISILTEKSRRFRKKLIERWACEIADFFIKNKVGTVQMEDLESMKRREDSYFNIRLRGFWPYAEMQSKIEFKLKQYGIEIRKVAPNNTSKTCSKCGHLNNYFNFEYRKKNKFPHFKCEKCNFKENADYNAALNISNPKLKSTKEEP

SEQ ID NO: 1169 - protein, 726 aa, synthetic construct
SEVEFSHEYWMRHALTLAKRARDEREVPVGAILVLNNRVIGEGWNRAIGLHDPTAHAEIMAMRQGGLVLQNYRLIDATLYVTFEPCVMCAGAMIHSRIGRVVFGVRNNKHGAAGSLVNVLNYPGMNHRVEITEGILADECAALLCDFYRMPRQVFNARKKAQSSINPGGSSGGSSGSETPGTSESATPESSGGSSGSSAKNTITKTLKLRIVRPYNSAEVEKIVADEKNNREKIALEKNKDKVKEACSKHLKVAAYCTTQVERNACLFCKARRLDDKFYQKLRGQFPDAVFWQEIGEIFRQLQKQAAEVYNQSLVELYYEILIKGKGIANASSVEHYLSDVCYTRAAELFKNAAIASGLRNKIKSNFRLKELRNMKSGLPTTKSDNFPIPLVRQKGGQYTGFEISNHDGDFIIKIPFGRWQVKKEINKHRPWEKFDFEQVRKSPKPISLLLSTQRRKRSKGWSKDEGTEAEIRKVMNGDYQTSYIEVKRGSKIGEKSAWMLNLSIDVPKIDKGVDPSIIGGIDVGVKSPLVCAINNALSRYSVSDNDLFHFNKKMFARRRILLRKNRHKRAGHGAKNKLKPITIMTEKSKRFRKKLIERWACEIADFFIKNKVGTVQMENLESMKRKEDSYFNIRLRGFWPYAEMQNKIEFKLKQYGIVVRKVAPNNTSKTCSKCGHLNNHFNFEYRKKNKFPLFKCEKCNFKENADYNAALNISNPKLKSTKGEP

SEQ ID NO: 1170 - protein, 726 aa, synthetic construct
SEVEFSHEYWMRHALTLAKRARDEREVPVGAVLVLNNRVIGEGWNRAIGLHDPTAHAEIMALRQGGLVMQNYRLTDATLYVTFEPCVMCAGAMVHSRIGRVVFGVRNSKRGAAGSLMNVLNYPDMNHYVEITEGILVDECAALLCDFYRMPRQVLNAQKKAQSSISSGGSSGGSSGSETPGTSESATPESSGGGSSGSAKNTITKTLQLRIVRPYNSAEVEKIVADEKNNREKIALEKNKDKVKEACSKHLKVASYCTTQVERDACPFCKARKLDDKFYQKLRGQFPDAVFWQELGEILRQLQKQAAEIYNQSLIELYYEIFIKGRGFANASSVEHYLSDVCYTRAAELFKNAAIASGLRGKVKSNFRLKELKNMKSGLPTTKSDNFPIPLVKQKGGQYTGFEISSHNDDFIIKIPFGRWQVKKEVDKYRPWEKFDFEQVRKSPKPISLLLSTQRRKRNKGWGKDEGTEAEIRKVMNGDYRTSYIEVKRGSKTGEKSAWMLSLSIDVPKIDKGVDPSIIGGIDVGVKSPLVCAINNAFSRYSISDNDLFRFNKKMFARRRILLKKNRHKRAGHGAKNKLKPISILTGKSERFRKKLIERWACEIADFFIKNKVGTVQMENLESMKRKEDSYFNIRLRGFWPYAEMQNRIEFKLKQYGIEIRKVAPNNTSKTCSKCGHLNNYFNFEYRKKNKFPHFKCEKCNFKENADYNAALNISNPKLKSTKEEP

SEQ ID NO: 1171 - protein, 726 aa, synthetic construct
SEVEFSHEYWMRHALTLAKRARDEREVPVGAVLVLNNRVIGEGWNRAIGLHDPTAHAEIMALRQGGLVMQNYRLIDATLYVTFEPCVMCAGAMVHSRIGRVVFGVRNSKHGAAGSLVNVLNYPGMNHRVEITEGILADECAALLCDFYRMPRQVFNARKKAQSSINPSGSSGGSSGSVTPGTSESATPESSGGGFGGSAKNTITKTLQLRIVRPYNSAEVEKIVADEKNNREKIALEKNKDKVKEACSKHLKVASYCTTQVERNACLFCKARKLDDKFYQKLRGQFPDAVFWQELGEIFRQLQKQAAEIYNQSLIELYYEIFIKGKGLANASSVEHYLSDVCYTRAAELFKNAAIASGLRGKVKSNFKLKELKSMKSGLPSTKSDNFPIPLVKQKGGQYTGFEISSHNDDFIIKIPFGRWQVKKEIDKYRPWEKFDFEQVRKSPKPISLLLSTQRRKRYKGWSKDEGTEAEIRKVMNGDYQTSYIEVKRGSKTGEKSAWMLNLSIDVPKIDKGVDPSIIGGIDVGVKSPLVCAINNAFSRYSISDNDLFHFNKKMFARRRILLRRNRHKRAGHGARNKLKPITVLTEKSERFRKKLIERWACEIANFFIKNKVGTVQMENLESMKRKEDSYFNIRLRGFWPYAEMQNKIEFKLKQYGIEIRKVAPNNTSKTCSRCGHLNNYFNFEYRKKNKFPHFKCEKCNFKEDADYNAALNISNPKLKSTKEEP

SEQ ID NO: 1172 - protein, 726 aa, synthetic construct
SEDEFSHEYWMRHALTLAKRARDGREVPVGAVLVLNNRVIGEGWNRAIGLHDPTAHAEIMALRQGGLVMQNYRLIDATLYVTFEPCVMCAGAMVHSRIGRVVFGVRNSKRGAAGSLMNVLNYPGMNHRVEITEGILADECAALLCDFYRMPRQVFNARKKARSNINSGGSSGGSSGSETLGTREGATPESSGGSSGGSAKNTITKTLKLRIVRPYNSAEVEKIVADEKNNREKIALEKNKDKVKEACSKHLKVASYCTTQVERNACPFCKARKLDDKFYQKLRGQFPDAVFWQELGEILRQLQKQAAEIYNQSLIELYYEIFIKGKGFANASSVEHYLSDVCYTRAAELFKNAAIASGLRGKVKSNFRLKELKNMKSGLPTTKSDNFPIPLVKQKGGQYTGFEISSHNDDFIIKIPFGRWQVKKEVDKYRPWEKFDFEQVRKSPKPISLLLSTQRRKRNKGWSKDEGTEAEIRKVMNGDYQTSYIEVKRGSKIGEKSAWMLNLSIDVPKIDKGVDPSIIGGIDVGVKSPLVCAINDAFSRYSISDNDLFHFNKKMFARRRILLKKSKHKRAGHGAKNKLKPITIMTEKSKRFRKKLIERWACEIADFFIKNKVGTVQMENLESMKRKEDSYFNIRLRGFWPYAEMQNKIEFKLKQYGIEVRKVAPNNTSRTCSKCGHLNNYFNFEYRRKNKFPHFKCEKCNFKENADYNAALNISDPKLKSTKEEP

SEQ ID NO: 1173 - protein, 726 aa, synthetic construct
SEVEFSHEYWMRHALTLARRARGEREVPVGAILVLNNRVIGEGWNRAIGLHDPTAHAEIMALRQGGLAMQNYRLTDATLYVTFEPCVMCAGAMIHSRIGRVVFGVRNSKHGAAGSLVNVLNYPGMNHRVEITEGILADECAALLCDFYRMPRQVFNARKKAQSSISSGGSSGGSSGSETPGASESVTPKSSVGSSAGSTKNTITKTLKLRIVRPYNSAEVEKIVADEKNNREKIALEKNKDKVKEACSKHLKVASYCTTQVERNACPFCKARKLDDKFYQKLRGQFPDAVFWQELGEILRQLQKQAAEIYNQSLIELYYEIFIKGRGFANASSVEHYLSDVCYTRAAELFKNAAIASGLRGKVKSNFRLKELKNMKSGLPTTKSDNFPIPLVKQKGGQYTGFEISSHNDDFIIKIPFGRWQVKKEIDKYRPWEKFDFEQVRKSPKPISLLLSTQRRKRNKGWSKDEGTEAEIRKVMNGDYQTSYIEVKRGSKIGEKSAWMLNLSIDVPKIDKGVDPSIIGGIDVGVKSPLVCAINNAFSRYSISDNDLFHFNKKMFARRRILLKKNRHKRAGHGAKNKLKPISILTEKSKRFRKKLIERWACEIADFFIKNKVGTVQMENLESMKRKEDSYFNIRLRGFWPYAEMQNKIEFKLKQYGIEIRKVAPNNTSKTCSKCGHLNNYFNFEYRKKNKFPHFKCEKCNFKENADYNAALNISNPRLKSTKEEP

SEQ ID NO: 1174 - protein, 726 aa, synthetic construct
SEVEFSHEYWMRHALTLAKRARDEREVPVGAVLVLNNRVIGVGWNRAIGLHDPTAHAEIMALRQGGLVTQNYRLIDATLYVTFEPCIMCAGAMIHSRIGRVVFGVRNSKRGAAGSLMNVLDYPGMNHRVEITEGILADECAALLCDFYRMPRQVFNAQKKARPNINSGGSSGGRSGSETPGTSESATPESSGGSSGGSAKNTITKTLKLRIVRPYNSAEVEKIVADEKNNREKIALEKNKDKVKEACSKHLKVAAYCTTQVERNACLFCKARKLDDRFYQKLRGQFPDAVFWQEIGEIFRQLQKQAAEIYNQSLIELYYEILIKGKGIANASSVEHYLSDVCYTRAAELFKNAAIASGLRGKVKSNFRLKELRSMKSGLPTTKSDNFPIPLVRQKGGQYTGFEISSHNDDFIIKIPFGRWQVKEEINKYRPWEKFDFEQVRKSPKPISLLLSTQRRKRNKGWSKDEGTEAEIRKVMNGDYQTSYIEVKRGSKIGEKSAWMLNLSIDVPKIDKGVDPSIIGGIDVGVKSPLVCAINNAFSRYSISDNDLFHFNKKMFARRRILLKKNRHRRAGHGAKNKLKPIAVLTEKSEGFRKKLIERWACEVADFFIKNKVGTVQMENLESMKRREDSYFNIRLRGFWPYAEMQNKIEFKLRQYGIEIRKVAPNNTSKTCSKCGHLNNYFDFEYRKKNKFPHFKCEKCNFKENADYNAALNISNPKLRSTKEEP

SEQ ID NO: 1175 - protein, 726 aa, synthetic construct
GEVEFSHEYWMRRALTLAKRARDEREVPVGAILVLNNRVIGEGWNRAIGLHDPTAHAEITALRQGGLVMQNYRLIDATLYVTFEPCVMCAGAMIHSRIGRVVFGVRNSKHGAAGSLVNVLNYPGMNHRVEITEGILADECAALLCDFYRMPRQVFIAQKKAQSTINSGGSSGGSSSSETPGTSGSATPEGSGGSSGGSAKNTITKTLKLRIVRPYNSAEVEKIVADEKNNREKIALEKNKDKVKEACSKHLKVASYCTTQVERNACLFCKARKLDDKFYQKLRGQFPDAVFWQELGEIFRQLQKQAAEIYNQSLIELYYEIFIKGKGFANASSVEHYLSDVCYTRAAELFKNAAIASGLRGKVKSNFRLKELKNMKSGLPTTKSDNFPIPLVKQKGGQYTGFEISNHNDDFIIKIPFGRWQVKEEIDRYRPWEKFDFEQVRKSPKPISLLLSTRRRKRNKGWSKDEGTEAEIRRVMNGDYQTSYIEVKRGSKIGEKSAWMLSLSIDVPKIDKGVDPRIIGGIDVGVKSPLVCAINNVPSRYSISDNDLFHFNKKMFARRRILLKKSRHKRAGHGTKNKLKPITILTEKSKRFRKKLIERWACEIADFFIKNKVGTVQMENLESMKRKEDSYFNIRLRGFWPYAEMQNKIEFKLKQYGIKIRKVAPNNTSKTCSKCGHLNNYFGFEYRRKNKFPHFKCEKCNFKEDADYNAALNISNPKLKSTKEEP

SEQ ID NO: 1176 - protein, 726 aa, synthetic construct
SEVEFSHEYWMRHALTLAKRARDEREVPVGAVLVLNNRVIGEGWNRAIGLHDPTAHAEIMALRQGGLVMQNYRLSDATLYVTFEPCVMCAGAMIHSRIGRVVFGARNGKRGAAGSLMNVLNYPGMNHCVEITEGILVDECAALLCDFYRMPRQVLSAQKKAQSSISSGGSSGGSSGSETPGASGSVTPKSSVGSSAGSTKNTITKTLKLRIVRPYNSAEVEKIVADEKNNREKIALEKNKDKVKEACSKHLKVAAYCTTQVERNACLFCKARKLDDKFYQKLRGQFPDAVFWQEISEIFRQLQKQAAEIYNQSLIELYYEIFIKGKGFANASSVEHYLSDVCYTRAAELFKNAAIASGLRGKVKSNFRLKELKNMKSGLPTTKSDNFPIPLVKQKGGQYTGFEISSHNDDFIIKIPFGRWQVKKEIDKYRPWEKFDFEQVRKSPKPISLLLSTQRRKRNKGWGKDEGTEAEIRKVMNGDYQTSYIEVKRGSKIGEKSAWMLSLSIDVPKIDKGVDPSIIGGIDVGVKSPLVCAINNAFSRYSISDNDLFHFNKKMFARRRILLKKNRHKRAGHGAKNKLKPISILTEKSGRFRKKLIERWACEIADFFIKNKVGTVQMENLEGMKRREDSYFNIRLRGFWPYAEMQNKIEFKLKQYGIKVRRVAPNNTSKTCSKCGHLNNYFSFEYRKKNKFPHFKCKKCNFKENADYNAALNISNPKLKSTREEP

SEQ ID NO: 1177 - protein, 726 aa, synthetic construct
NEVEFSHEYWMRHALTLAKRARDEREVPVGAVLVLNNRVIGEGWNRTTGLHDPTAHAEIMALRQGGLVMQNHRLVDATLYVTFEPCVMCAGAMIHSRIGRVVFGVRNSKRGAAGSLTNVLNYPGMNHRVEITEGILADECAALLCDFYRMPRQVFNARKKAQSSINPGGPSGGSSGSKTPGTSESVTPKSSGGSSAGSTKNTITKTLKLRIVRPYNSAEVEKIVADEKNSREKIALERNKDKVKEACSEHLKVAAYCTTQVERNACLFCKARKLDDRFYQKLRGQFPDAVFWQETGEIFRQLQRQAAEIYNQSLIELYYEIFIKGKGFANASSVEHYLSDVCYTRAAELFKNAAIASGLRGKVKSNFRLKELKNMKSGLPTTKSDNFPIPLVKQKGGQYTGFEISSHNDDFIIKIPFGRWQVKKEIDRYRPWEKFDFEQVRKSPKPISLLLSTRRRKRNKGWSKDEGTEAEIRKVMNGDYLTSYIEVKRGSKIGEKSAWMLNLSIDVPKIDKGVDPSIIGGIDVGVKSPLVCAINNASSRYSISDNDLFRFNKKMFARRRILLKKNRHKRAGHGAKNKLKPISILTGKSERFRKKLIERWACEIADFFIKNKVGTVQMENLESMKRKEDSYFNIRLRGFWPYAEMQNKIEFKLKQYGIEIRKVAPNNTSKTCSKCGHLNNYFNFEYRKKNKFPHFKCEKCNFKENADYNAALNISNPKLKSTKEEP

SEQ ID NO: 1178 - protein, 726 aa, synthetic construct
SEVEFSHEYWMRHALTLAKRARDEREVPVGAVLVLNNRVIGEGWNRAIGLHDPTAHAEIMALRQGGLVMQNYRLTDATLYVTFEPCVMCAGAMIHSRIGRVVFGVRNSKRGAAGSLMNVLNYPGMNHCVEITEGILVDECAALLCDFYRMPRQVLNAQKKAQSSISPGGSSGGSSGSETPGASGSVTPKSSGGSSAGSTKDTITKTLKLRIVRPYNSAEVEKIVADEKNSREKIALEKYKDKVKEACSEHLKVAAYCTTQVERNACLFCKARKLDDRFYQKLRGQFPGAVFWQEIGEIFRQLQKQAAEIYNQSLIELYYEIFIKGKGFANASSVEHYLSDVCYTRAAELFKNAAIASGLRGKVKSNFRLKELKNMKSGLPTTKSDNFPIPLVRQKGGQYTGFEISNHNGDFIIKIPFGRWQVKKEINKHRPWEKFDFEQVRKSPKPISLLLSTQRRKRNKGWGKDEGTEAEIRKVMNGDYQTSYIEVKRGSKIGEKSAWMLNLSIDVPKIDKGVDPSIIGGIDVGVKSPLVCAINNAFSRYSISDNDLFRFNKKMFARRRILLRKNRHKRAGHGAKNKLKPITIMTEKSKRFRKKLIERWACEIADFFIKNKVGTVQMENLESMKRKVDSYFNVRLRGFWPYAEMQNKIEFRLKQYGIEVRKVAPNNTSKTCSKCGHLNNYFNFEYRKKNKFPHFKCEKCNFKEDADYNAALNISNPKLKSTKGEP

SEQ ID NO: 1179 - protein, 726 aa, synthetic construct
SEVEFSHEYWMRHALTLAKRARDEREVPVGAVLVLNNRVIGEGWNRAIGLHDPTAHAEIMALRQGGLVLQNYRLVDATLYVTFEPCVLCAGAMVHSRIGRVVFGARNSKRGAAGSLMNILNYPGMNHRVEITEGILADECAALLCDFYRMPRRVFNARKKAQSSIDPGGPSGGSSGNETPGTSESATPESSGGSSGGSAKNTITKTLKLRIVRPYNSTEVEKIVADEKNNREKVALEKNKDKVKEACSKHLKVASYCTTQVERNACLFCKARKLDDKFYQKLRGQFPDAVFWQELGEIFRQLQKQAAEIYNQSLIELYYEIFIKGKGFANASSVEHYLSDVCYTRAAELFKNAAIASGLRGKVKSNFRLKELKNMKSGLPTTKSDNFPIPLVKQKGGQYTGFEISSHNDDFIIKIPFGRWQVKKEIDKYRPWEKFDFEQVRKSPKPISLLLSTQRRKRNKGWSKDEGTEAEIRKVMNGDYQTSYIEVKRGSKIGEKSAWMLNLSIDVPKIDKGVDPSIIGGIDVGVKSPLVCAINNAFSRYSISDNDLFHHNKKMFARRRILLKKNRHKRAGHGAKDKLKPISILTEKSKRFRKKLIERWACEIADFFIKNKVGTVQMENLESMKRKEDSYFNIRLRGFWPYAEMQNKIEFKLKQYGIEIRKVAPNNTSKTCSKCGHLNNYFNFEYRKMNKFPHFKCEKCNFKENADYNAALNISNPKLKSTKEEP

SEQ ID NO: 1180 - protein, 726 aa, synthetic construct
SEVEFSHEYWMRHALTLAKRARDEREVPVGAILVLNNRVIGVGWNRAIGLHDPTAHAEIMALRQGGLVMQNYRLIDATLYVTFEPCVMCAGAMIHSRIGRVVFGVRNSKHGAAGSLVNVLNYPGMNHRVEITEGILADECAALLCDFYRMPHQVFNARKRAQSSINSGGSSGSSSGSETPGTSESATPKSSGGSSGGSAKNTITKALKLRIVRPYNSAEVEKIVADEKNNREKIALEKNKDKVREACSKHLKVASYCTTQVERNACPFCKARKLDDKFYQKLRGQFPDAVFWQEISEIFRQLQKQAAEVYNQSLVELYYEILIKGKGIANASSVEHYLSDVCYTRAAELFKNAAIASGLRNKIKSNFRLKELRNMKSGLPTTKSDNFPIPLVKQKGGQYTGFEISNHNSDFIIKIPFGRWQAKKEIDKYRPWEKFDFEQVRKSPKPISLLLSTQRRKRNKGWSKDEGTEAEIEKVMNGDYQTSYIEVKRGSKTGEKSTWMLNLSIDVPKIDKGVDPRIIGGIDVGVKSPLVCAINNVLSRYSISDNDLFHFNKKMFARRRILLKKNGHKRAGHGAKNKLKPITIMTEKSKRFRKKLIERWACEIADFFIKNKVGTVQMENLESMKRKEDSYFNIRLRGFWPYAEMQNKIEFKLKQYGIVVRKVAPNNTSKTCSQCGHLNNYFNFEYRKKNKFPHFKCEKCNFREDADYNAALNISNPELKSTKEES

SEQ ID NO: 1181 - protein, 726 aa, synthetic construct
SEVEFSHEYWMRHALTLAKRARDEREVPVGAVLVLNNRVIGEGWNRAIGQHDPTAHAEIMALRQGGLVMQNYRLIDATLYVTFEPCVMCAGAMVHSRIGRVVFGVRNSKRGAAGSLMNVLDYPGMGHRVEITEGILADECAALLCDFYRMPRQVFNAQKRAQSSINSGGSSGGSSGSETPGASESVTPKSSGGSSGGSAKNTITKTLKLRIVRPYNSAEVEKIVADEKNNREKIALEKNKGKVKEACSKHLEVAAYCTTQVERNACLFCKARKLDDKFYQKLRGQFPDAVFWQELGEIFRQLQKQAAEIYNQSLIELYYEIFIKGKGFANASSVEHYLSDVCYTRAAELFKNAAIASGLRGKVKSNFRLKELKNMKSGLPTTKSDNFPIPLVKQKGGQYTGFEISSHNDDFIIKIPFGRWQVKKEIDKYRPWEKFDFEQVRKSPKPISLLLSTQRRKRNKGWSKDEGTEAEIRKVMNGDYQTSYIEVKRGSKIGEKSAWMLNLSIDVPKIDKGVDPSIIGGIDVGVKSPLVCAINNAFSRYSISDNELFHFNKKMFARRRILLKKNRHKRAGHGAKNKLRPISILTEKSERFRKKLIEKWACEIADFFIKNKVGTVQMENLESMKRKEDSYFNIRLRGFWPYAEMQNKIEFKLKQYGIEIRKVAPYNTSKTCSKCGHLNYYFNFEYRKKNKFPHFKCEKCNFKENADYNAALNISNPKLKSTKEEP

SEQ ID NO: 1182 - protein, 726 aa, synthetic construct
SEVEFSHEYWMRHALILAKRARDEREVPVGAVLVLNNRVIGVGWNRAIGLHDPTAHAEIMALRQGGLVMQNYRLSDATLYVTFEPCVMCAGAMIHSRIGRVVFGVRNSKRGAAGSLMNVLNYPGMNHCVEITEGILVDECAALLCDFYRMPRQVLSAQKKAQSSVSSGGSSGGSSGSETPGASGSVIPRSSGGSSAGSTKDTITKTLKLRIVRPYNSAEVEKVVADEKNNREKIAMEKNKDKVREACSKHLKVASYCTTQVERNACLFCKARKLDDKFYQKLRGQFPDAVFWQELGGIFRQLQKQAAEIYNQSLIELYYEIFIKGKGITNASRVEHYLSDVCYTRAAELFKNAAIASGLRSKVRSNFRLKELKNMKSGLPTTKSDNFPIPLVKQKGGQYTGFEISSHNSDFIIKIPFGRWQEKEEIDKYRPWEKFDFEQVRRSPKPISLLLSTQRRKKNKGWSKDEGTEAEIRRVMNGDYQTSYIEVKRGSKIGEKSAWMLNLSIDVPKIDKGVDPSIIGGIDVGVKSPLVCAINNAFSRYSISDNDLFRFNKKMFARRRILLKKNRHKRAGHGAKNKLKPISILTGKSERFRKKLIERWACEIADFFIKNKVGTVQMENLESMKRKEDSYFNIRLRGFWPYAEMQNKIEFKLKQYGIEIRKVAPNNTSKTCSKCGHLNNYFNFEYRKKNKFPHFKCEKCNFKENADYNAALNISNPKLKSTKEEP

SEQ ID NO: 1183 - protein, 726 aa, synthetic construct
SEVEFSHEYWMRHALTLAKRARDEREVPVGAVLVLNNRVIGVGWNRAIGLHDPTAHAEIMALRQGGLVMQNYRLTDATLYVTFEPCVMCAGAMVHSRIGRVVFGVRNSKRGAAGSLMNVLNFPGMSHCVEITEGILVDECAALLCDFYRMPRRVFNAQKKAQSSINSGGSSGGGSGSEMPGASESVTPKSSGGSSAGSTKNTITKTLKLRIVRPYNSAEVEKIVADEKNSREKIALERNKDKVKEACSKHLKVAAYCTTQVERNACLFCKARRLDDKFYQKLRGQFPDAVFWQEIGEIFRQLQKQAAETYNQSLIELYYEIFIKGKGIANASNVEHYLSDVCYTRAAELFKNAAIASGLRNKIKSNFRLKELRNMKSGLPTTKSDNFPIPLVKQKGGQYTGFEISNHNGDFIIKIPFGRWQAKKEIDKYRPWEKFDFEQVRKSPKPISLLLSTQRRKRNRGWSKDEGTEAEIKKVMNGDYQTSYIEVKRGNKIGEKSAWMLNLSIDVPKISKGVDPSIIGGIDVGVKSPLVCAINNTFSRYSISDNDLFHFNKKMFARRRILLKKSKHKRAGHGAKNKLKPITILTEKSGRFRKKLIERWASEIADFFIKNKVGTVQMENLESMKRKEDSYFNIRLRGFWPYAEMQNKIEFKLKQYGIEVRKVAPNNTSKTCSKCGHLNNYFNFEYRKKNKFPHFRCEKCNFKENADYNAALNISNPKLKSTKEEP

SEQ ID NO: 1184 - protein, 726 aa, synthetic construct
SEVEFSHEYWMRHALALAKRARDEREVPVGAVLVLNNRAIGEGWNRAIGLHDPTAHAEIMALRQGGLVMQNYRLTDATLYVTFEPCVMCAGAMIHSRIGRVVFGVRNSKRGAAGSLMNVLNYPGMNHYVEITEGILVDECAALLCDFYRMPRQVLNAQKKAQSSISSGGSSGGSSGSETPGASESATPKSSGGSSAGSTKNTITKTLKLRIVRPYNSAEVEKIVADEKNNRERIALEKNKDKVKEACSKHLKVAAYCTTQVERNACLFCKARKLDDKFYQKLRGQFPDAVFWQETGEIFRQLQRQAAEIYNQSLIELYYEIFIKGKGFANASSVEHYLSDVCYTRAAELFKNAAIASGLRGKVKGNFRLKELKNMKSGLPTTKSDNFPIPLVKQKGGQYTGFEISSHNDDFIIKIPFGRWQAKKEIDKYRPWEKFDFEQVRKSPKPISLLLSTQRRKRNKGWSKDEGTEAEIRKVMNGDYQTSYIEVKRGSKIGEKSAWMLNLSIDVPKIDKGVDPSIIGGIDVGVKSPLVCAINNAFSRYSISDNDLFHFNKKMFARRRILLKKNRHKRAGHGAKNKLRPITILAEKSERFRKKLIEKWACEIADFFIKNKVGTVQMENLESMKRKEDSYFNIRLRGFWPYAEMQNKIEFKLKQYGIEIRKVAPNNTSKTCSKCGHLNNYFNFEYRKKNKFPHFKCEKCNFKENADYNAALNISNPKLKSTKEEP

SEQ ID NO: 1185 - protein, 726 aa, synthetic construct
SEVEFSHEYWMRHALTLAKRARDEREVPVGAVLVLNNRVIGEGWNRTTGLHDPTAHAEIMALRQGGLVMRNYRLTDATLYVTFEPCVMCAGAMIHSRIGRVVFGVRNSKRGAAGSLMNVLNYPGMNHCVEITEGILVDECAALLCDFYRMPRQVLNAQKKAQSSISPGGSSGGSSDSETPGASESVTPKSSGGSSGGSAKNTITKTLKLRIVRPYNSAEVEKIVADEKNSREKIALEKNKGKVKEACSKHLEVAAYCTTQVERNACLFCKARKLDDKFYQKLRGQFPDAVFWQELGEIFRQLQKQAAEIYNQSLIELYYEIFIKGKGFANAGSVEHYLSNVCYTRAAELFKNAAIASGLRGKVKSNFRLKELKSMKSGLPTTKSDNFPIPLVKQKGGQYTGFEISSHNDDFIIKIPFGRWQVKKEIDKYRPWEKFDFEQVRKSPKPISLLLSTQRRKRNKGWSKDEGTEAEIRKVMNGDYQTSYIEVKRGSKIGEKSAWMLNLSIDVPKIDKGVDPSIIGGIDVGVKSPLVCAINNAFSRYSIGDNDLFHYNKKMFARRRILLKKNRHKRAGHGAKNKLKPISILTEKSKRFRKKLIERWACEIADFFIKNKVGTVQIENLESMKRKEDSYFNIRLRGFWPYAEMQNKIEFKLKQYGIEIRKVAPNNTSKTCSKCGHLNSYFNFEYRKKNKFPYFKCEKCNFKENADYNAALNISNPKLKSTKEEP

SEQ ID NO: 1186 - protein, 726 aa, synthetic construct
SEVEFSHEYWMRHALTLAKRARDEREVPVGAVLVLNNRVIGEGWNRAIGLHDPTAHAEIMALRQGGLVMQNYRLTEATLYVTFEPCVMCAGAMIHSRIGRVVFGVRNSKRGAAGSLMNVLNYPGMNHCVEITEGILVDECAALLCDFYRMPRQVLNAQKKAQSSISSGGSSGGSSGSEMPGASESVTPKSSGGSSGGSAKNTITKTLKLRIVRPYNSAEVEKIVADEKNNREKIALEKNKDKVKEACSKHLKVAAYCTTQVERNACLFCKARKLDDKFYQKLRGQFPDAVFWQEISEIFRQLQKQAAEIYNQSLIELYYEIFIKGKGFANASSVEHYLSDVCYTRAAELFKNAAIASGLRGKVKSNFRLKELKNMKSGLPTTKSDNFPIPLVKQKGGQYTGFEISSHNDDFIIKIPFGRWQVKKEIDKYRPWEKFDFEQVRKSPKPISLLLSTQRRKRNKGWSKDEGTEAEIRKVMNGDYQTSYIEVKRGSKIGEKSAWMLNLSIDVPKIDKGVDPSIIGGIDVGVKSPLVCAINNALSRYSISDNDLFHFNKKMFARRRILLKKNRHRRAGHGTKNKLKPISILTEKSKRFRKKLIERWACEIADFFIKNKVGTVQMENLESMKRKEDSYFNIRLRGFWPYAEMQNKIEFKLKQYGIEIRKVAPINTSKTCSKCGHLNNYFNFEYRKKNKFPHFKCEKCNFKENADYNAALNISNPMLRNTKEEP

SEQ ID NO: 1187 - protein, 726 aa, synthetic construct
SEVEFSHEYWMRHALTLAKRARDEREVPVGAVLVLNNRVIGVGWNRAIGLHDPTAHAEIMALRQGGLVMQNYRLTDATLYVTFEPCVMCAGAMVHSRIGRVVFGVRNSKRGAAGSLMNVLNYPGMSHCVEITEGILVDECAALLCDFYRMPRQVLNAQKKAQSSISSGGSSGGSSGSETPGASESVTPKSSVGSSAGSTKNTITKTLKLRIVRPYNSAEVEKIVADEKNNREKIALEKNKDKVKEACSRHLKVAAYCTTQVERNACLFCKARKLDDKFYQKLRGQFPDAVFWQELGEIFRQLQKQAAEIYNQSLIELYYEIFIKGKGFANASSVEHYLSDVCYTRAAELFKNAAIASGLRGKVKSNFRLKELKNMKSGLPTTKSDNFPIPLVKQKGGQYTGFEISSHNSDFIIKIPFGRWQVKEEIDKYRPWEKFDFEQVRKSPKPISLLLSTQRRKKNKGWSKDEGTEAEIRRVMNGDYQTSYIEVKRGSKIGEKSAWMLNLSIDVPKIDKGVDPSIIGGIDVGVKSPLVCAINNSFSRYSICDNDLFRFNKKMFARRRILLKKNRHKRAGHGAKNKLKPITILTKKSERFRKKLIERWVCEVADFFIKNKVGTVQMENLESMKRKEDSYFNIRLRGFWPYAEMQNRIEFKLKQYGIEIRKVAPNNTSKTCSKCGHLNNYFNFEYRKKNKFPHFKCEKCNFKENADYNAALNISNPKLKSTKEEP

SEQ ID NO: 1188 - protein, 726 aa, synthetic construct
SEGEFSHEYWMRHALTLAKRARDGREVPVGAVLVLNNRVIGEGWNRAIGLHDPTAHAEIMALRQGGLVMQNYRLIDATLYVTFEPCVMCAGAMVHSRIGRVVFGVRNSKRGAAGSLMNVLDYPGMGHRVEITEGILVDECAALLCDFYRMPRQVLNAQKKAQSSISSGGSSGGSSGSETPGASGSVIPKSSGGSSAGSTKDTITKTLKLRIVRPYNSAEVEKIVADEKNNREKVALEKNKDKVKEACSEHLRVAAYCTTQVERNACLFCKARKLDDKFYQKLRGQFPDAVFWQEIGEIFRQLQKQAAEIYNQSLIELYYEIFIKGKGFANASSVEHYLSDVCYARAAELFKNAAIASGLRGKVKSNFRLKELKNMRSGLPTTKSDNFPIPLVKQKGGQYTGFEISSHNDDFIIKIPFGRWQVKKEIDKYRPWEKFDFEQVRKSPKPISLLLSTQRRKRNKGWSKDEGTEAEIRKVMNGDYQTSYIEVKRGSKIGEKSTWMLSLSIDVPKIDKGVDPSIIGGIDVGVKSPLVCAINNACSRYSISDNDLFHFNKKMFARRRILLKKNRHKRAGHGAKNKLKPITILTEKSKRFRKKLIERWACEIADFFIKNKVGTVQMENLESMKRKEDSYFNTRLRGFWPYAEMQNKIEFKLKQYGIEIRKVAPNDTSKTCSKCGHLNNYFNFEYRKKNKFPHFKCEKCSFKENADYNAALNISNPKLKSTKEEP

SEQ ID NO: 1189 - protein, 726 aa, synthetic construct
SEAEFSHEYWMRHALTLAKRARDEREVPVGAVLVLNNRVIGEGWNRAIGLHDPTAHAEIMALRQGGLVMQNYRLTDATLYVTFEPCVMCAGAMIHSRIGRVVFGVRNGKRGAAGSLMNVLNYPGMNHCVEITEGILVDECAALLCDFYRMPRQVLNAQKKAQSSISSGGSSGGSSGSETPGASESTTPESSGGSSGGPAKNTITKTLKLRIVRPYNSAEVEKIVADEKNNREKTALEKNKDKVKEACSKHLKVAAYCTTQVERNACLFCKARKLDDKFYQKLRGQFPDAVFWQEVGEIFRQLQKQAAEIYNQSLIELYYEIFIKGKGFANASSVEHYLSDVCYTRAAELFKNAAIASGLRGKVKSNFRLRELKNMKSGLPTTKSDNFPIPLVKQKGGQYTGFEISNHNSDFIIKIPFGRWQVKKEINKYRPWEKFDFEQVRKSPKPISLLLSTQRRKRNKGWSKDEGTEAEIRKVMNGDYQTSYIEVKRGSRIGEKSAWMLSLSIDVPKIDKGVDPSIIGGIDVGVKSPLVCAINNALSRYSISDNDLFHFNKKMFARRRILLKRNRHKRAGHGAKNKLKPITILTEKSKRFRRKLIERWACEIADFFIKNKVGTVQMENLEGMKRREDSYFNIRLRGFWPYAEMQNKIEFKLKQYGIEVRKVAPNNTSKTCSKCGHLNNYFNFEYRKKNKFPHFKCEKCNFKENADYNAALNISNPKLKSTKEEP

SEQ ID NO: 1190 - protein, 726 aa, synthetic construct
SEVEFSHEYWMRHALTLAKRARDEREVPVGAVLVLNNRVIGEGWNRAIGLHDPTAHAEIMALRQGGLVMQNYRLIDATLYVTFEPCVMCAGAMIHSRIGRVVFGVRNNKRGAAGSLMNVLNYPGMNHRVEITEGILADECAALLCDFYCMPRQVLNAQKKARSCINSGGSSGGSSGSETPGTSESATPESSGGGSSGSAKNTITKTLQLRIVRPYNSAEVEKIVADEKNNREKIALEKNKDKVKEACSKHLKVASYCTTQVERNACPFCKARKLDGKFYQKLRGQFPDAVFWQELGEILRQLQKQAAEIYNQSLIELYYEIFIKGRGFANASSVEHYLSDVCYTRAAELFKNAAIASGLRGKVKSNFRLKELKNMKSGLPTTKSDNFPIPLVKQKGGQYTGFEISSHNDDFIIKIPFGRWQVKKEIDKYRPWEKFDFEQVRKNPKPISLLLSTQRRKRNKGWSKDEGTEAEIKKVMNGDYQTSYIEVKRGSKTGEKSAWMLNLSIDVPKIDKGVDPSIIGGIDVGVKSPLVCAINNAFSRYSISDNDLFRFNKKMFARRRILLRKNRHKRAGHGAKNKLKPISILTGKSERFRKKLIERWACEIADFFIKNKVGTVQMENLESMKRKEDSYFNIRLRGFWPYAEMQSKIEFKLKQYGIEIRKVAPNNTSKTCSKCGHLNNYFNFEYRKRNKFPHFKCEKCNFKENADYNAALNISNPKLKGTKEEP

SEQ ID NO: 1191 - protein, 726 aa, synthetic construct
SEVEFSHEYWMRHALALAKRARDEREVPVGAVLVLSNRAIGEGWNRAIGLHDPTAHAEIMALRQGGLVMQNYRLTDATLYVTFEPCVMCAGAMIHSRIGRVVFGVRNSKRGAAGSLMNVLNYPGMNHCVEITEGILVDECAALLCDFYRMPRQVLNAQKKAQSSISSGGSSGGSSGSETPGASGSVTPKSSGGGFGSSAKNTITKTLQLRIVRPYNSAEVEKIVADEKNNREKIALEKNKDKVKEACSEHLKVAAYCTTQVERNACLFCKARKLDDKFYQKLRGQFPDAVFWQELGEIFRQLQKQAAEIYNQSLIELYYEIFIKGKGFANASSVEHYLSDVCYTRAAELFKNAAIASGLRGKVKSNFRLKELKNMKSGLPTTKSDNFPIPLVKQKGGQYTGFEISSHNDDFIIKIPFGRWQVRKEIDKYRPWEKFNFEQVRKSPKPISLLLSTQRRKRNKGWSKDEGTEAEIRKVMNGDYQTSYIEVKRGSKIGEKSAWMLNLSIDVPKIDKGVDPSIIGGIDVGVKSPLVCAINNSSSRYSICDNDLFRFNKKMFARRRILLKKNRHKRAGHGAKNKLKPITVLTEKSKRFRKKLIERWACEIANFFIKNKVGTVQMENLESMKRKEDSYFNIRLRGLWPYAEMQNKIEFKLKQYGIEVRKVAPNNTSKTCSKCGHLNNYFNFEYRKRNKFPHFKCEKCNFKENADYNAALNISNPKLKGTKEEP

SEQ ID NO: 1192 - protein, 726 aa, synthetic construct; identical to SEQ ID NO: 1093

SEQ ID NO: 1193 - protein, 726 aa, synthetic construct
SEVEFSHEYWMRHALTLAKRARDEREVPVGAVLVLNNRVIGEGWNRTTGLHDPTAHAEIMALRQGGLVMRNYRLTDATLYVTFEPCAMCAGAMIHSRIGRVVFGVRNSKRGAAGSLMNVLNYPGMNHCVEITEGILVDECAALLCDFYRMPRRVFNARKKAQSSIDPGGPSGGSSGSETPGTSESATPESSGGSSGGSAKNTITKTLKLRIVRPYNSTEVEKIVADEKNNREKIALEKNKDKVKEACSKHLKVASYCTTQVERNACLFCKARKLDDKFYQKLRGQFPDAVFWQEISEIFRQLQKQAAEIYNQSLIELYYEIFIKGKGFANASSVEHYLSDVCYTRAAELFKNAAIASGLRGKVKSNFRLKELKNMKSGLPTTKSDNFPIPLVKQKGGQYTGFEISSHNDDFIIKIPFGRWQAKKEIDKYRPWEKFDFEQVRKSPKPISLLLSTQRRKRNRGWSKDEGTEAEIRKVMNGDYQTSYIEVKRGSKIGEKSAWMLSLSIDVPKIDKGVDPSIIGGIDVGVKSPLVCAINNAFSRYSISDNDLFRFNKKMFARRRILLKKNRHKRAGHGVKNKLKPISILTEKSERFRKKLIERWACEIADFFIRNKVGTVQMENLEGMKRKEDSYFNIRLRGFWPYAEMQNKIEFKLKQYGIVVRKVAPNDTSKTCSKCGHLNNYFNFEYRKKNKFPHFKCEKCNFKENADYNAALNISNPKLKSTKEEP

SEQ ID NO: 1194 - protein, 726 aa, synthetic construct
SEVEFSHEYWMRHALTLAKRARDEREVPVGAVLVLNNRVIGEGWNRAIGLHDPTAHAEIMALRQGGLVMQNYRLTDATLYATFEPCVMCAGAMIHSRIGRVVFGVRNSKRGAAGSLMNVLNYPGMNHCVEITEGILVDECAALLCDFYRMPRQVFNAQKKAQSTINSGGSSGGSSGSETPGTSESPTPESSGGSPGGSAKNTITKTLKLRIVRPYNSAEVEKIVADEKNNREKIALEKNKDKVKEACSKHLKVASYCTTQVERNACPFCKARKLDDKFYQRLRGQFPDAVFWQELGEILRQLQKQAAEIYNQSLIELYYEIFIKGRGFANASSVEHYLSDVCYTRAAELFKNAAIASGLRGKVKSNFRLKELKNMKSGLPTTKSDNFPIPLVKQKGGQYTGFEISSHNDDFIIKIPFGRWQVKKEIDKYRPWEKFDFEQVRKSPKPISLLLSTQRRKRNKGWSKDEGTEAEIKKVMNGDYQTSYIEVKRGSKTGEKSAWMLNLSIDVPKIDKGVDPCIIGGIDVGVKSPLVCAINNALSRYSISDNDLFHFNKKMFARRRILLRKNRHKRAGHGAKNKLKPISVLTGKSERFRKKLIERWACEIADFFIKNKVGTVQMENLESMKRKEDSYFNIRLRGFWPYAEMQNKIEFKLKQYGIVVRKVAPNNTSKTCSQCGHLNNYFDFEYRKKNKFPYFKCEKCNFKENADYNAALNISNPQLKSTKGEP

SEQ ID NO: 1195 - protein, 726 aa, synthetic construct
SEVEFSHEYWMRHALTLAKRARDEREVPVGAILVLNNRVIGEGWNRAIGLHDPTAHAEIMALRQGGLVMQNYRLIDATLYVTFEPCVMCAGAMIHSRIGRVVFGVRNSKHGAAGSLVNVLNYPGMNHRVEITEGILADECAALLCDFYRMPHQVFGARRKAQSSINPGGSSGGSSGSETPGASESVTPKSSVGSSAGSTKNTITKTLKLRIVRPYNSAEVEKIVADEKDNRERIALEKNKDKVKEACSKHLMVASYCTTQVERSACLFCKARELDGRFYQKLRGQFPDAVFWQEIGEIFRQLQKQAAEIYNQSLIELYYEIFIKGKGFANASSAEHYLSDVCYTRAAELFKNAAIASGLRGKVKSNFRLKELKNMKSGLPTTKSDNFPIPLVKQKGGKYTGFEISSHNDDFIIKIPFGRWQVKKEIDRYRPWEKYDFEQVRKSPKPISLLLSTQRRKRNKGWSKDEGTEAEIRKVMSGDYQTSYIEVKRGSKVGEKSAWMLNLSIDVPKIDKGVDPSIVGGIDVGVKSPLVCAINNAFSRYSISDNDLFRFNKKVFARRRILLKKNRHKRAGHGTKNKLKPISILTEKSKRFRKKLIERWACEIADFFIKNKVGTVQMENLESMKRKEDSYFNIRLRGFWPYAEMQNKIEFKLKQYGIEIRKVAPNNTSKTCSKCGHLNNYFNFEYRKKNKFPHFKCEKCNFKEDADYNAALNISNPKLKSTKEEP

SEQ ID NO: 1196 - protein, 726 aa, synthetic construct
NEVEFSHEYWMRHALTLAKRARDEREVPVGAVLVLNNRVIGEGWNRTTGLHDPTAHAEIMALRQGGLVMQNYRLIDATLYVTFEPCVMCAGAMIHSRIGRVVFGVRNNKHGAAGSLVNVLNYPGMNHRVEITEGILADECAALLCDFYRMPRQVFNARKKTQSSINPGGSSGGSSGSETPGTSVSATPESSGSSSGGSAKNTITKTLKLRIVRPYNSAEVEKIVADEKNNREKIALEKNKDKVKEACSKHLKVATYCTTQVERSACLFCKARRLDDKFYQKLRGQFPDAVFWQEIGEIFRQLQKQAAEIYNQSLVELYYEIFIKGKGIANASSVEHYLSGVCYTRAAELFKNAAIASGLRNKVKSNFRLKELRNMKSGLPTTKSDNFPIPLVRQKGGQYTGFEISNHNSDFIIKIPFGRWRVKKEIDKYRPWEKFDFAQVRKSPKPISLLLSTQRRKRNRGWSKDEGTEAEIKKVMNGDYQTSYIEVKRGSKIGEKSAWMLNLSIDVPKIDKGVDPSIIGGIDVGVKSPLVCAINNAFSRYSISDNDLFHFNKKMFARRRILLKKNRHKRAGHGAKNKLKPISILTEKSKRFRKKLIERWACEIADFFIKNKVGTVQMENLESMKRKEDSYFNIRLRGFWPYAEMQNKIEFKLKQYGIEIRKVAPNNTSKTCSKCGHLNNYFNFEYRRKNKFPHFKCEKCNFKEDADYNAALNISNPKLKSTKEEP

SEQ ID NO: 1197 - protein, 726 aa, synthetic construct
SEVEFSHEYWMRRALTLAKRARDEREVPVGAVLVLNNRVIGVGWNRAVGLHDPTAHAEIMALRQGGLVMQNYRLIEATLYVTFEPCIMCAGAMIHSRIGRVVFGVRNSKRGAAGSLMNVLNYPGMNHRVEITEGILVDECAALLCDFYRMPRQVLNAQKKAQSSISPGGSSGGSSGSETPDASGSVTPKSSGGSSAGSTKDTITKTLQLRIVRPYNSAEVEKIVADEKNNREKIALEKNKDKVKEACSKHLKVASYCTTQVERNACLFCKARKLDDKFYQKLRGQFPDAVFWQELGEIFRQLQKQAAEVYNQSLIELYYEIFIKGRGFANASSVEHYLSDVCYTRAAELFKNAAIASGLRGKVKSNFRLKELKNMKSGLPTTKSDNFPIPLVKQKGGQYTGFEISSHNDDFIIKIPFGRWQVKKEIDKYRPWEKFDFEQVRKSPKPISLLLSTQRRKRNKGWSKDEGTEAEIRKVMNGDYQTSYIEVKRGSKIGEKSAWMLNLSINVPKIDKGVDPSIIGGIDVGVKSPLVCAVNNALSRYSISDNDLFHFNKKMFARRRILLKKNRHKRAGHGAKNKLKPITILTEKSVRFRKKLIERWACGIADFFVKNKVGTVQMENLESMKRREDSYFNIRLRGFWPYAEMQSKIEFKLKQYGIKIRKVAPNNTSKTCSKCGHLNNYFNFEFRKKNKFPHFKCEKCNFKEDADYNAALNISDPKLKGTKEEP

SEQ ID NO: 1198 - protein, 726 aa, synthetic construct
SEVEFGHEYWMRHALTLAKRARDEREVPVGAILVLNNRVIGEGWNRAIGLHDPTAHAEIMALRQGGLVMQNYRLIDATLYVTFEPCVMCAGAMIHSRIGRVVFGVRNSKHGAAGSLVNVLNYPGMNHRVEITEGILADECAALLCDFYRMPRQVFNARKKAQSTINSGSSSGGSSGSETPGTSESPTPESSGGIPGGSAKNTITKTLKLRIVRPYNSAEVEKIVADEKNNREKIALEQNKDKVREACSKHLKVAAYCTTQVERNACLFCKARRLDDKFYQKLRGQFPDAVFWQEIGEIFRQLQKQAAEIYNQSLIELYYEIFIKGKGFANASSVEHYLSDVCYTRAAELFKNAAIASGLRGKVKSNFRLKELKNMKSGLPTTKSDNFPIPLVKQKGGQYTGFEISNHNDDFIIKIPFGRWQVKKEIDKYRPWEKFDFEQVRKSPKPISLLLSTQRRKRNKGWSKDEGTEAEIRKVMNGDYQTSYIEVKRGSRIGEKSAWMLSLSIDVPKIDRGVDPSIIGGIDVGVKSPLVCAINNALSRYSISDNDLFHFNKKMFARRRILLKKNRHRRAGHGARNKLKPITVLTEKSKRFRKKLIERWACEIADFFIKNKVGTVQMENLESMKRKEDSYFNIRLRGLWPYAEMQNKIEFKLKQYGIEIRKVAPNNTSKTCSKCGHLNNYFNFEYRKRNKFPHFKCEKCNFKENADYNAALNISSPKLKSTKEGP

SEQ ID NO: 1199 - protein, 726 aa, synthetic construct
SEVEFSHEYWMRHALTLAKRARDEREVPVGAVLVLNNRVIGEGWNRAIGLHDPTAHAEIMALRQGGLVMQNYRLIDATLYVTFEPCVMCAGAMVHSRIGRVVFGVRNSKRGAAGSLMNVLNYPGVNHCVEITEGILVDECAALLCDFYRMPRHVLNAQKKAQSSINSGGSSGGSSGSETPGTSESATPESSGGGSSGSAKNTITKTLQLRIVRPYNSAEVEKIVADEKNNREKIALEKNKDKVKEACSKHLKMASYCTTQVERNACLFCKARKLDDKFYQKLRGQFPDAVFWQELGGIFRQLQKQAAEIYNQSLIELYYEIFIKGKGITNASRVEHYLSDVCYTRAAELFKNAAIASGLRSKVRSNFRLKELKNMKSGLPTTKSDNFPIPLVKQKGGQYTGFEISSHNSDFIIKIPFGRWQVKEEIDKYRPWEKFDFEQVRKSPKPISLLLSTQRRKKNKGWSKDEGTEAEIRRVMNGDYQTSYIEVKRGSKIGEKSAWMLNLSIDVPTIDKGVDPSIIGGIDVGVKSPLVCAINNAFSRYSISDNDLFRFNKKVFARRRILLKKNRHKRAGHGAKNKLKPISILTEKSERFRKKLIERWACEIADFFIRNKVGTVQMENLEGMKRKEDSYFNIRLRGFWPYAEMQNKIEFKLKQYGIEVRKVAPNNTSKTCSKCGHLNNYFNFEYRKKNKFPHFKCEKCNFKENADYNAALNISNPKLKSTKEEP

SEQ ID NO: 1200 - protein, 726 aa, synthetic construct
SEVEFSHEYWMRHALTLAKRARDEREVPVGAVLVLNNRVIGEGWNRAIGLHDPTAHAEIMALRQGGLVMQNYRLIDATLYVTFEPCVMCAGAMVHSRIGRVVFGVRNSKRGAAGSLMNVLDYPGMGHRVEITEGILADECAALLCDFYRMPRQVFNAQKRAQSSINSGGSSGGSSGSETPGTSESPTPESSGGSPGGSAKNTITKTLKLRIVRPYNSAEVEKIVADEKNNREKIALEKNKDKVKEACSKHLKVAAYCTTQVERNACLFCKARKLDDKFYQKLRGQFPDAVFWQEIGEIFRQLQKQAAEIYNQSLIELYYEIFIKGKGFANASSVEHYLSDVCYTRAAELFKNAAIASGLRGKVKSNFRLKELKNMKSGLPTTKSDNFPIPLVKQKGGQYTGFEISSHDDDFIIKIPFGRWQVKEEIVKYRPWEKFDFEQVRKSPKPISLLLSTQRRKRNKGWSKDEGTEAEIRKVMNGDYQTSYIEVKRGSKVGEKSAWMLNLSIDVPKIDKGVDPSIVGGIDVGVKSPLVCAINNAFSRYSISDNDLFHFNKKMFARRRILLRKSKHKRAGHGAKNKLKPITILTEKSGRFRKKLIERWACEIADFFIKNKVGTVQMENLESMKRKEDSYFNIRLRGFWPYAEMQNKIEFKLKQYGIEIRKVAPNNTSKTCSKCGHLNNYFNFEYRKKNKFPHFKCEKCNFKENADYNAALNISNPKLKSTKEEP

SEQ ID NO: 1201 - protein, 726 aa, synthetic construct
SEVEFSHEYWMRHALTLAKRARDEREVPVGAVLVLNNRVIGEGWNRAIGLHDPTAHAEIMALRQGGLVMQNYRLSDATLYVTFEPCVMCAGAMIHSRIDRVVFGVRNSKRGAAGSLMNVLNYPGMNHCVEITEGILVDECAALLCDFYRMPRQVLSAQKKAQSSISSGGSSGGSSGSETPGASGSVTPKSSVGSSAGSTKNTITKTLKLRIVRPYNSAEVEKIVADEKNNREKIALEKNKDKVKEACSKHLKVASYCTTQVERNACLFCKARKLDDGFYQKLRGQFPDAVFWQELGEIFRQLQKQAAEIYNQSLIELYYEIFIKGKGITNASRVEHYLSDVCYTRAAELFKNAAIASGLRGKVKSNFRLKELKNMKSGLPTTKSDNFPIPLVKQKGGQYTGFEISSHNDDFIIKIPFGRWQVKEEIDKYRPWEKFDFEQVRKSPKPISLLLSTQRRKKNKGWSKDEGTEAEIRRVMNGDYQTSYIEVKRGSKIGEKSAWMLNLSIDVPKIDKGVDPSIIGGIDVGVKSPLVCAINNSFSRYSICDNDLFRFNKKMFARRRILLKKNRHKRAGHGAKNKLKPITILTKKSERFRKKLIERWVCEVADFFIKNKVGTVQMENLESMKRKEDSYFNIRLRGFWPYAEMQSKIEFKLKQYGIKVRKVAPNNTSKTCSKCGHLNNYFNFEFRKKSKFPHFKCEKCNFKEDADYNAALNISNPKLKGTKEEP

SEQ ID NO: 1202 - protein, 726 aa, synthetic construct
SEVEFSHEYWMRHALTLAKRARDEREVPVGAVLVLNNRVIGEGWNRAIGLHDPTAHAEIMALRQGGLVMQNYRLTDATLYVTFEPCVMCAGAMIHSRIGRVVFGVRNSKRGAAGSLMNVLNYPGMNHCVEITEGILVDECAALLCDFYRMPRQVLNAQKKAQSSISSGGSSGGSSGSKTPGARGSVTPKSSGGGSAGSTKDTITKTLKLRIVRPYNSAEVEKIVADEKNSREKIALEKNKDKVKEACSEHLKVAAYCTTQVERNACLFCKARKLDDKFYQRLRGQFPDAVFWQEIGEIFRQLQKQAAEIYNQSLIELYYEIFIKGKGFANASSVEHYLSDVCYTRAAELFKNAAIASGLRGKVKSNFRLKELKNMKSGLPTTKSDNFPIPLVKQKGGQYTGFEINSHNDDFVIKIPFGRWRVKKEIDKYRPWEKFDFEQVRKSPKPISLLLSTQRRKRNKGWSKDEGTEAEIRKVMNGDYQTSYIEVKRGSKIGEKSAWMLNLSIGVPKIDKGVDPSIIGGIDVGVKSPLVCAINNAFSRYSISDNDLFHFNKKMFARRRILLKKNRHKRAGHGAKNKLKPISILTERSKRFRKKLIERWACEIADFFIKNKVGTVQMENLESMKRKEDSYFNIRLRGFWPYAEMQNKIEFKLKQYGIEIRKVAPNNTSKTCSKCGHLNNYFNFEYRRMNKFPHFKCEKCNFKENADYNAALNISNPKLKSTKEEP

SEQ ID NO: 1203 - protein, 726 aa, synthetic construct
SEVEFSHEYWMRHALTLANRARDEREVPVGAILVLNNRVIGEGWNRAIGLHDPTAHAEIMALRQGGLVMQNYRLIDATLYVTFEPCVMCAGAMVHSRIGRVVFGVRNSKRGAAGSLMNVLDYPGMGHRVEITEGILADECAALLCDFYCMPRQVFNAQKRAQSSINSGGSSGGSSGSETPGTSESATPESSGGGSSGSAKNTITKTLQLRIVRPYNSAEVEKIVADEKNNREKIALEKNKDKVREACSKHLKVAAYCTTQVERNACLFCKARRLDDKFYQKLRGQFPDAVFWQEIGEIFRQLQKQAAVIYNQSLIELYYEIFIKGKGIANASSVEHYLSDVCYTRAAELFKNAAIASGLRNKVKSNFRLKELKSMKSGLPTTKSDNFPIPLVRQKGGQYTGFEISNHNSDFIIKIPFGRWQAKKEIDKYRPWEKFDFEQVRKSPKPISLLLSTQRRKRNKGWNKDEGTEAEIRKVMNGDYQTSYIEVKRGSKIGEKSAWMLNLSIDVPKIDKGVDPSIIGGIDVGVKSPLVCAINNAFSRYSISDNDLFRFNKKMFARRRILLKKNRHKRAGHGAKNKLKPISILTGKSERFRKKLIERWACEIADFFIKNKVGTVQMENLESMKRKEDSYFNIRLRGFWPYAEMQNKIEFKLKQYGIEIRKVAPNNTSKTCSRCGHLNNYFNFEYRKKNKFPHFKCEKCNFKENADYNAALNISNPKLKSTKEKP

SEQ ID NO: 1204 - protein, 726 aa, synthetic construct
SEVEFSHEYWMRHALTLAKRARDEREVPVGAVLVLNNRIIGEGWNRAIGQHDPTAHAEIMALRQGGLVMQNYRLTDATLYVTFEPCVMCAGAMVHSHIGRVVFGVRNSKRGAAGSLMNVLNYPGVNHCVEITEGILVDECAALLCDFYRMPRRVFNAQKKAQSSINSGGSSGGGSGSETPSTSESTTPESSGGGSSGSAKNTITKTLQLRIVRPYNSAEVEEIVADEKNNREKIALEKNKDKVKEACSKHLKVAAYCTTQVERNACLFCKARKLDDKFYQKLRGQFPDAVFWQEIGEIFRQLQKQAAEIYNQSLIELYYEIFIKGKGFANASSVEHYLSDVCYTRAAELFKNAAIASGLRGKVKSNFRLKELKNMKSGLPTTKSDNFPIPLVKQKGGQYTGFEISSHHDDFIIKIPFGRWQVKKEIDKYRPWEKFDFEQVRKSPKPISLLLSTQRRKRNKGWSKDEGTEAEIRKVMNGDYQTSYIEVKRGSKIGEKSAWMLSLSIDVPKIDKGVDPSIVGGIDVGVKSPLVCAINNALGRYSISDNDLFHFNKKMFARRRILLKKNRHKRAGHGAKNKLKPITILTEKSKRFRKKLIERWACEIADFFIKNKVGTVQMENLESMKRKEDSYFNIRLRGFWPYAEMQNKIEFKLKQYGIEIRKVAPNNTSKTCSKCGHLNNYFNFEYRKKNKFPHFKCEKCNFKESADYNAALNISNPKLKSTKEEP

SEQ ID NO: 1205 - protein, 726 aa, synthetic construct; identical to SEQ ID NO: 684

SEQ ID NO: 1206 - protein, 726 aa, synthetic construct
SEVEFSHEYWMRHALTLAKRARDEREVPVGAILVLNNRVIGEGWNRAIGLHDPTAHAEIMALRQGGLVMQNYRLIDATLYVTFEPCVMCAGAMIHSRIGRVVFGVRNNKHGAAGSLVNVLNYPGMNHRVEITEGILADECAALLCDFYRMPRRVFNAQKKAQSSINSGGSSGGSSGSVTPGTSESATPESSGGGSSGSAKNTITKTLQLRIVRPYNSAEVEKIVADEKNNREKIALEKNKDKVKEACSKHLKVASYCTTQVERNACPFCKARKLDDKFYQKLRGQFPDAVFWQEIGEIFRQLQKQAAEIYNQSLIELYYEIFIKGKGFAIASSVEHYLSCVCYTRAAELFKNAAIASGLRGKVKSNFRLKELKNMKSGLPTTKSDNFPIPLVKQKGGQYTGFEISSHNDDFIIKIPFGRWQVKKEIDKYRPWEKFDFEQVRKSPKPISLLLSTQRRKRNKGWSKDEGTEAEIRKVMNGDYQTSYIEVKRGSKIGEKSAWMLNLSIDVPKIDKGVDPSIVGGIDVGVKSPLVCAIDNALSRYSISDNDLFHFNKKMFARRRILLKKNRHRRAGHGAKNKLKPISILTEKSKRFRKKLIERWACEIADFFIKNKVGTVQMENLESMKRKEDSYFNIRLRGFWPYAEMQNKIEFKLKQYGIEIRKVAPNNTSKTCSKCGHLNNYFNFEYRKKNKFPHFKCEKCNFKENADYNAALNISNPMLKSTKEEP

SEQ ID NO: 1207 - protein, 726 aa, synthetic construct
SEAESSHEYWMRHALTLAKRARDEREVPVGAILVLNNRVIGEGWNRAIGLHDPTAHAEIMALRQGGLVMQNYRLIDATLYVTFEPCVMCAGAMIHSRIGRVVFGVRNNKHGAAGSLVNVLNYPGMNHCVEITEGILVDECAALLCDFYRMPRQVLSAQKKAQSSISSGGSSGGSSGSETPGASGSVTPRSSVGSSAGSTKNTITKTLQLRIVRPYNSAEVEKIVADEKNNREKIALEKNKDKVKEACSKHLKVASYCTTQVERNACLFCKARKLDDKFYQKLRGQFPDAVFWQELGEIFRQLQKQAAEIYNQSLIELYYEIFIKGRGFANASSVEHYLSDVCYTRAAELFKNAAIASGLRGKVKSNFRLKELRNMKSGLPTTKSDNFPIPLVKQKGGQYTGFEISSHNDDFIIKIPFGRWQVKKEIDKYRPWEKFDFEQVRKSPKPISLLLSTQRRKRNKGWSKDEGTEAEIRKVMNGDYQTSYIEVKRGSKTGEKSTWMLNLSIDVPKIDKGVDPSIIGGIDVGVKSPLVCAINNAFSRYSISDNDLFRFNKKMFARRRILLKKNRHKRAGHGAKNKLKPITILTKKSERFRKKLIERWACEIADFFIKNKVGTVQMENLESMKRKEDSYFNIRLRGFWPYAEMQNKIEFKLKQYGIEIRKVAPNNTSKTCSKCGHLNNYFNFEYRKRSKFPHFKCEKCNYREDADYNAALNISNPKLKSTKEEP

SEQ ID NO: 1208 - protein, 726 aa, synthetic construct
SEVEFSHEYWMRHALTLAKRARDEREVPVGAVLVLNNRVIGEGWNRAIGLHDPTAHAEIMALRQGGLVMQNYRLTDATLYVTFEPCVMCAGAMIHSRIGRVVFGVRNSKRGAAGSLMNVLNYPGMNHCVEITEGILAGECAALLCDFYRMPRQVFNARKKAQSSINSGGSSDGGSGSETPGTCESVTPESSGGSSGGSAKNTITKTLKLRIVRPYNSAEVEKVVADEKNNREKIAMEKNKDKVKEACSKHLKVASYCTTQVERNACLFCKARKLDDKFYQKLRGQFPDAVFWQEIGEIFRQLQKQAAEIYNQSLIELYYEIFIKGKGVANASSVEHYLSDVCYTRAAELFKNAAIASGLRNKVKSNFRLKELRSMKSGLPTTKSDNFPIPLVRQKGGQYTGFEISNHNSDFTIKIPFGRWQAKKEIDKYRPWEKFDFEQVRKSPKPISLLLSTQRRKRNKGWSKDEGTEAEIRKVMNGDYQTSYIEVKRGSKVGEKSAWMLNLSIDVPKIDKGVDPSIIGGIDVGVKSPLVCAVNNALSRYSISDNDLFHFNKKMFARRRILLRKNRHKRAGHGAKNKLKPITMMTEKSKRFRKKLIERWACEIADFFIKNKVGTVQMENLESMKRKEDSYFNIRLRGFWPYAEMQNKIEFKLKQYGIEIRKVAPNNTSKTCSKCGHLNNYFNFEYRKKNKFPHFKCEKCNFKENADYNAALNISNPRLKSTKEEP

SEQ ID NO: 1209 - protein, 726 aa, synthetic construct
SEVEFSHEYWMRHALTLAKRARDEREVPVGAVLVLNNRVIGEGWNRTTGLHDPTAHAEIMALRQGGLVMQNHRLVDATLYVTFEPCVMCAGAMIHSRIGRVVFGVRNGKRGAAGSLTNVLNYPGMNHRVEITEGILVDECAALLCDFYRMPRQVFNAQKKAQSTINSGGSSGGSSGSETPGTSESPTPESSGGSPGGSAKNTITKTLKLRIVRPYNSAEVEKIVADEKNNREKIALEKNKDKVKEACSKHLKVAAYCTTQVERNACLFCKARKLDDKFYRELRGQFPDAVFWQELGEIFRQLQKQAAEIYNQSLIELYYEIFIKGKGFANASSVEHYLSDVCYTRAAELFKNAAIASGLRGKVKSNFRLKELKNMKSGLPTTKSDNFPVPLVKQKGGQYTGFEISSHNDDFIIKIPFGRWQVKEEIDKYRPWEKFDFEQVRKSPKPISLLLSTQRRKKNKGWSKDEGTEAEIRRVMDGDYQTSYIEVKRGSKIGEKSAWMLSLSIDVPKIDKGVDPSIIGGIDVGVKSPLVCAINNAFCRYSISDNDLFHFNKKMFARRRILLKKSRHKRAGHGAKNKLKPISILTEKSKRFRKKLIERWACEIADFFIKNKVGTVQMENLESMKRKEDSYFNIRLRGFWPYAEMQNKIEFKLKQYGIEIRKVAPNNTSKTCSKCGHLNNYFNFEYRKMNKFPHFKCEKCNFKENADYNAALNISNPKLKSTKEEP

SEQ ID NO: 1210 - protein, 726 aa, synthetic construct
SEVEFSHEYWMRHALTLAKRARDEREVPVGAVLVLNNRVIGEGWNRAIGLHDPTAHAEIMALRQGGLVMQNYRLTDATLYVTFEPCVMCAGAMIHSRIGRVVFGVRNSKRGAAGSLMNVLNYPGMNHCVEITEGILVDECAALLCDFYRMPRQVLNAQKKAQSSINPSGSSGGSSGSVTPGTSESATPESSGGGFGGSAKNTITKTLQLRIVRPYNSAEVEKIVADEKNNREKIALEKNKDKVKEACSKHLKVASYCTTQVERNACLFCKARKLDDKFYQKLRGQFPDAVFWQELGEIFRQLQKQAAEIYNQSLVELYYEILIKGKGIANASSVEHYLSDVCYTRAAELFKNAAIASGLRNKIKSNFRLKELRNMKSGLPTTKSDNFPIPLVRQKGGQYTGFEISNHDGDFIIKIPFGRWQVKKEINKHRPWEKFDFEQVRKSPKPISLLLSTQRRKRNKGWSKDEGTEAEIRKVMNGDYQTSYIEVKRGSKIGEKSAWMLNLSIDVPKIDKGVDPGIIGGIDVGVKSPLVCAINNASSRYSISDNDLFHFNKKMFARRRILLKKNRHKRAGHGAKNKLKPITIMTEKSKRFRKKLIERWACEIADFFIKNKVGTVQMENLESMKRKEDSYFNIRLRGFWPYAEMQNKIEFKLKQYGIEIRKVAPNNTSKTCSKCGHLNNYFNFEYRKKNKFPHFKCEKCNFKENADYNAALNISNPKLKSTKEEP

SEQ ID NO: 1211 - protein, 726 aa, synthetic construct
SEVEFSHEYWMRHALALAKRARDEREVPVGAVLVLNNRAIGEGWNRAIGLHDPTAHAEIMALRQGGLVMQNYRLTDATLYVTFEPCVMCAGAMIHSRIGRVVFGVRNSKRGAAGSLMNVLNYPGMNHYVEITEGILADECAALLCDFYRMPRQVFNARKKAQSSINPGGSSGGSSGSETPGTSESATPESSGGSSGSSAKNTITKTLKLRIVRPYNSAEVEKIVADEKNNREKIALEKNKDKVKEACSKHLKVAAYCTTQVERNACLFCKARRLDDKFYQKLRGQFPDAVFWQEIGEIFRQLQKQAAEVYNQSLVELYYEILIKGKGIANASSVEHYLSDVCYTRAAELFRNAAIASGLRNKIKSNFRLKELRNMKSGLPTTKSDNFPIPLVRQKGGQYTGFEISNHDGDFIIKIPFGRWQVKEEIDKYRPWEKFDFEQVRKSPKPISLLLSTQRRKKNKGWSKDESTEAEIRRVMNGDYQTSYIEVKRGSKIGEKSAWMLNLSIDVPKIDKGVDPSIIGGIDVGVKSPLVCAINNSSSRYSICDNDLFRFNKKMFARRRILLKKNRHKRAGHGAKNKLKPITILTKKSERFRKKLIERWVCEVADFFIKNKVGTVQMENLESMKRKEDSYFNIRLRGFWPYAEMQNRIELKLKQYGIEIRKVAPNNTSKTCSKCGHLNNYFNFEYRKKNKFPHFKCEKCNFKENADYNAALNISNPKLKSTKEEP

SEQ ID NO: 1212 - protein, 726 aa, synthetic construct
SEVEFSHEYWMRHALTLAKRARDEREVPVGAILVLNNRVIGEGWNRAIGLHDPTAHAEIMALRQGGLVMQNYRLVDATLYVTFEPCVLCAGAMVHSRIGRVVFGVRNSKRGAAGSLMNVLNHPGMNHRVEITEGILADECAALLCDFYRMPRQVFNARKKAQSSINPDGSSGGSGGSETPGTSESPTPESSGGSSGGSAKNTITKTLKLRIVRPYNSAEVEKIVAEEKDNREKIALEKNKDKVREACSKHLRVAAYCTTQVERNACLFCKARKLDDKFYQKLRDQFPDAVFWQEIGEIFRQLQKQAAEIYNQSLIELYYEIFIKGKGFANASSVEHYLSDVCYTRAAELFKNAAIASGLRGKVKSNFRLKELKNMKSGLPTTKSDNFPIPLVKQKGGQYTGFEISSHNDDFIIKIPFGRWRVKKEIGKYRPWEKFDFEQVRKSPKPISLLLSTQRRKRNRGWSKDEGTEAEIRKVMNGDYQTSYIEVKRGSKIGEKSAWMLNLSIDVPKIDKGVDPSIIGGIDVGVKSPLVCAINNAFSRYSISDNDLFRFNKKMFARRRILLKKNRHKRAGHGAKNKLKPITILTGKSRRFRKKLIERWACEIADFFIKNKVGTVQMESLESMKRKEDSYFNIRLRGFWPYAEMQNKIEFKLKQYGIKIRKVAPNNTSKTCSKCGHLNNYFSFEYRKKNKFPHFKCEKCNFKENADYNAALNISNPKLMSTKEEP

SEQ ID NO: 1213 - protein, 726 aa, synthetic construct
SEVEFSHEYWMRRALTLAKRARDEREVPVGAVLVLNNRVIGEGWNRAIGLHDPTAHAEIMALRQGGLAMQNYRLVDATLYVTFEPCVLCAGAMVHSRIGRVVFGVRNSKRGAAGSLMNVLNHPGMNHRVEITGGILADECAALLCDFYRMPRQVFNVRKKARSNINSGGSSGGSSGSETLGTSESATPESSGGSSGGSAKNTITKTLKLRIVRPYNSAEVEKIVADEKNNREKIALEKNKDKVKEACSKHLKVASYCTTQVERNACLFCKARKLDDKFYQKLRGQFPDAVFWQELGEIFRQLQKQAAEIYNQSLIELYYEIFIKGKGIANASSVEHYLSDVCYTRAAELFRNAAIASGLRNKIKSNFRLKELRNMKSGLPTTKSDNFPIPLVRQKGGQYTGFEISNHNGDFIIKIPFGGWQVKKEISKHRPWEKFDFEQVRKSPKPISLLLSTQRRKRNKGWGKDEGTEAEIRKVMNGDYQTSYIEVKRGSKIGEKSAWMLNLSIDVPKIDKGVDPSIIGGIDVGVKSPLVCAINNALGRYSISDNDLFHFNKKMFARRRILLRKNRHKRAGHGVRNKLKPITVLTEKSERFRKKLIERWACEIANFFIKNKVGTVQMENLESMKRREDSYFNIRLRGFWPYAEMQSKIEFKLKQYGIKIRKVAPNNTSKTCSKCGHLNNYFNFEFRKKNKFPHFKCEKCNFKEDADYNAALNISNPKLKSTKEEP

SEQ ID NO: 1214 - protein, 726 aa, synthetic construct
SEVEFSHEYWMRRALTLAKRARDEREVPVGAVLVLNNRVIGVGWNRAVGLHDPTAHAEIMALRQGGLVMQNYRLIEATLYVTFEPCIMCAGAMIHSRIGRVVFGVRNSKRGAAGSLMNVLNYPGMNHRVEITEGILADECAALICDYYRMPRQVFNARKKAQSSINSGGSSGGSSGSETPSTSESATPESSGGSSGGSAKNTITKTLQLRIVRPYNSAEVEKIVTDEKNNREKIALEKNKDKVKEACSKHLKMASYCTTQVERNACLFCKARKLDDKFYQKLRGQFPDAVFWQETGEIFRQLQRQAAEIYNQSLIELYYEIFIKGKGFANASSVEHYLSDVCYTRAAELFKNAAIASGLRGKVKGNFRLKELKNMKSGLPTTKSDNFPIPLVKQKGGQYTGFEISSHNDDFIIKIPFGRWQAKKEIDKYRPWEKFDFEQVRRSPKPISLLLSTQRRKRNKGWSKDEGTEAEIRKVMNGDYQTSYIEVKRGSKIGEKSVWMLNLSIDVPKIDRGVDPSIIGGIDVGVKSPLVCAINNAFSRYSISDNDLFHFNKKMFARRRILLKKNRHKRAGHGAKNKLKPITIMTEKSKRFRKKLIERWACEIADFFIKNKVGTVQMENLESMKRKEDSYFNIRLRGFWPYAEMQNKIEFKLKQYGIEIRKVAPNNTSKTCSKCGHLNYYFNFEYRKKNKFPHFKCEKCNFKEDADYNAALNISNPKLKSTKEEP

SEQ ID NO: 1215 - protein, 726 aa, synthetic construct
SEVEFSHEYWMRHALTLAKRARDEREVPVGAILVLNNRVIGEGWNRAIGLHDPTAHAEIMALRQGGLVMQNYRLIDATLYVTFEPCVMCAGAMIHSRIGRVVFGVRNNKHGAAGSLVNVLNYPGMNHRVEITEGILADECAALLCDFYRMPRQVLNAQKKAQSSISSGGSSGGSGGGETPGASESVTPKSSGGSSAGSTKNTITKTLKLRIVRPYNSAEVEKIVADEKNSREKIALEKNKDKVKEACSEHLKVAAYCTTQVERSACLFCKARKLDDRFYQKLRGQFPDAVFWQEIGEIFRQLQKQAAEVYNQSLVELYYEILIKGKGIANASSVEHYLSDVCYTRAAELFKNAAIASGLRNKIKSNFRLKELRNMKSGLPTTKSDNFPIPLVKQKGGQYTGFEISSHNSDFIIKIPFGRWQVKEEIDKYRPWEKFDFEQVRKSPKPISLLLSTQRRKRNKGWGKDEGTEAEIRRVMNGDYQTSYIEVKRGSKIGEKSAWMLNLSIDVPKIDKGVDPRIIGGIDVGVKSPLVCAINNAFSRYSISDNDLFRFNKKMFARRRILLGKNRHKRAGHGVKNKLKPITILTEKSGRFRKKLIERWACEIADFFIKNKVGTVQMENLESMKRKEDSYFNIRLRGFWPYAEMQNKIEFKLKQYGIVVRKVAPNNTSKTCSQCGHLNNYFNFEYRKKNKFPYFKCEKCNFKENADYNAALNISNPQLKSTKGEP

SEQ ID NO: 1216 - protein, 726 aa, synthetic construct
SEVEFSHEYWMRHALTLAKRARDEREVPVGAVLVLNDRVIGEGWNRAIGLHDPTAHAEIMALRQGGLVMQNYRLTDATLYVTFEPCVMCAGAMIHSRIGRVVFGVRNSKRGAAGSLMNVLNYPGMNHCVEITEGILVDECAALLCDFYRMPRQVLNAQKKAQPSISSGGSSGGSSGSETPGASGSVTPKSSGGSSAGSTKDTITKTLKLRIVRPYNSAEVEKIVADEKDNREKIALEKNKDKVKEACSKHLKVAAYCTTQVERNACLFCRARKLDDGFYQKLRGQFPDAVFWQEIGEIFRQLQKQAAEIYNQSLIELYYEIFIKGKGFANASSVEHYLSDVCYTRAAELFKNAAIASGLRGKVKSNFRLKELKNMKSGLPTTKSDNFPIPLVKQKGGQYTGFEISSHNDDFIIKIPFGRWQAKKEIDKYRPWEKFDFERVRKSPKPISLLLSTQRRKRNKGWSKDEGTEAEIEKVMNGDYQTSYIEVKRGSKTGGKSAWMLNLSIDVPKIDKGVDPCIIGGIDVGVKSPLVCAINDAFSRYSISDNDLFHFNKKMFARRRILLKKNGHKRAGHGAKNKLKPITIMTEKSKRFRKKLIERWACEIADFFIKNKVGTVQMENLESMKRKEDSYFNIRLRGFWPYAEMQNKIEFKLKQYGIEIRKVAPNNTSKTCSRCGHLNNYFNFEYRRKNKFPHFKCEKCNFKENADYNAALNISNPKLKSTKEEP

SEQ ID NO: 1217 - protein, 726 aa, synthetic construct
SEVEFSHEYWMRHALTLAKRARDEREVPVGAVLVLNNRVIGEGWNRAIGLHDPTAHAEIMALRQGGLVLQNYRLVDATLYVTFEPCVLCAGAMVHSRIGRVVFGARNSKRGAAGSLMNILNYPGMNHRVEITEGILADECAALLCDFYRMPRQVFNAQKKAQSSINPGGSSGGSSGSETPGTSESATPESSGGSSGSSAKNTITKTLKLRIVRPYNSAEVEKIVADEKNNREKIALEKNKDKVREACSKHLKVASYCTTQVERNACLFCKARKLDDRFYQKLRGQFPDAVFWQELGEIFRQLQKQAAEIYNQSLIELYYEIFIKGKGFANASSVEHYLSDVCYTRAAELFKNAAIASGLRGKVKSNFRLKELKNMKSGLPTTKSDNFPIPLVKQKGGQYTGFEISSHNDDFIIKIPFGRWQVKKEIDKYRPWEKFDFEQVRKSPKPISLLLSTQRRKRNKGWSKDEGTEAEIRKVMSGDYQTSYIEVKRGSKTGEKSAWMLNLSIDVPKIDKGVDPSIIGGIDVGVKSPLVCAINNAFSRYSISDNDLFRFNKKMFARRRILLKKNRHKRVGHGAKNKLKPISILTGKSERFRKKLIERWACEIADFFIKNKVGTVQMENLESMKRKEDSYFNIRLRGFWPYAEMQNKIEFKLKQYGIEIRKVVPNNTSKTCSKCGHLNNYFNFEYRKKNKFPHFKCEKCNFKENADYNAALNISNPKLKSTKEEP

SEQ ID NO: 1218 - protein, 726 aa, synthetic construct
NEVEFSHEYWMRHALTLAKRARDEREVPVGAVLVLNNRVIGEGWNRTTGLHDPTAHAEIMALRQGGLVMQNHRLVDATLYVTFEPCVMCAGAMIHSRIGRVVFGVRNSKRGAAGSLTNVLNYPGMGHRVEITEGILADECAALLCDFYRMPRQVFNAQKRAQSSINSGGSSGGSSGSETPGTSESATPESSGGGSSGSAKNTITKTLKLRIVRPYNSAEVEKIVADEKNNREKIALEKNKDKVKEACSKHLKVAAYCTTQVERNACLFCKARRLDDKFYQKLRGQFPDAVFWQEIGEIFRQLQKQAAEIYNQSLIELYYEIFIKGKGFANASSVEHYLSDVCYTRAAELFKNAAIASGLRGKVKSNFRLKELKSMKSGLPTTKSDNFPIPLVKQKGGQYTGFEISSHNDDFIIKIPFGKWQEKKEINKYRPWERFDFEQVRKSPKPISLLLSTQRRKRNKGWGKDEGTEAEIKKVMNGDYQTSYIEVKRGSKIGEKGAWMLNLSIDVPKIDKGVDPSIIGGIDVGVKSPLVCAINNAFSRYSISDNDLFRFNKKMFARRRILLKKNRHKRAGHGARNKLKPITILTEKSERFRKKLIERWACEIADFFIKNKVGTVQMENLESMKRKEDSYFNIRLRGFWPYAEMQNKIEFKLKQYGIEIRKVAPNNTSKTCSKCGHLNNYFNFEYRKMNKFPHFKCEKCNFKEDADYNAALNISNPKLKSTKEEP

SEQ ID NO: 1219 - protein, 726 aa, synthetic construct
SEVEFSHEYWMRHALTLAKRARDEREVPVGAVLVLNNRVIGVGWNRAIGLHDPTAHAEIMALRQGGLVLQNYRQTDATLYVTFEPCVMCAGAMIHSRIGRVVFGVRNSKRGAAGSLMNVLNYPGMSHRVEITEGILADECAALLCDFYHMPRQVFSAQKKAQSSINSGGSSGGSSGSETPGTSESATPKSSGGSSGGSAKNTITKALKLRIVRPYNSAEVEKIVADEKNSREKIALERNKDKVKEACSEHLKVAAYCTTQVERNACLFCKARKLDDRFYQKLRGQFPDAVFWQETGEIFRQLQRQAAEIYNRSLIELYYEIFIKGKGFANASSVEHYLSDVCYTRAAELFKNAAIASGLRGKVKSNFRLKELKNMKSGLPTTKSDNFPIPLVKQKGGQYTGFEISSHNDDFIIKIPFGRWQVKKEIDKYRPWEKFDFEQVRKSPKHISLLLSTQRRKRNKGWSKDEGTEAEIKKVMNGDYQISYIEVKRGSKIGEKSAWMLNLSVDVPKIDKGVDPSIIGGIDVGVKSPLVCAINNAFSRYSISDNDLFHYNKKMFARRRILLKKNRHKRAGHGAKNKLKPISILTEKSKRFRKKLIERWACEIADFFIKNKVGTVQIENLEGMKRKEDSYFNIRLRGFWPYAEMQNKIEFKLKQYGIEIRKVAPNNTSKTCSRCGHLNSYFNFEYRKKNKFPHFKCKKCSFKENADYNAALNISNPKLKSTKEEP

SEQ ID NO: 1220 - protein, 726 aa, synthetic construct
SEVEFSHEYWMRHALTLAKRARDEREVPVGAVLVLNNRVIGEGWNRAIGLHDPTAHAEIMALRQGGLVMQNYRLSDATLYVTFEPCVMCAGAMIHSRIGRVVFGVRNNKHGAAGSLVNVLNYPGMNHRVEITEGILADECAALLCDFYRMPRQVFNARKKAQSSINSGGSSGGSSGSETPGTSESATPKNSGGSSGGSAKNTITKALKLKIVRPYNSAEVEKIVADEKNYRERIALEKNKDKVKEACSKHLKVAAYCTTQVERNACLFCKARRLDDKFYQKLRGQFPDAVFWQEIGEIFRQLQKQAAEIYNQSLVELYYEILIKGKGFANASSVEHYLSDVCYTRAAELFKNAAIASGLRGKVKSNFRLKELKNMKSGLPTTKSDNFPIPLVKQKGGQYTGFEISSHNDDFIIKIPFGRWQVKKEIDKYRPWEKFDFEQVRKSPKPISLLLSTQRRKRNKGWSKDEGTEAEIRRVMNGDYQTSYIEVKRGSKIGEKSAWMLNLSIDVPKIDKGVDPSIIGGIDVGVRSPLVCAIDNAFSRYSISDNDLFHFNKKMFARRRILLKKNRHKRAGHGAKNKLKPISILTEKSKRFRKKLIERWACEIADFFIKNKVGTVQMENLESMKRKEDSYFNIRLRGLWPYAEMQNKIEFKLKQYGIEIRKVAPNNTSKTCSKCGHLNNYFNFEYRKKNKFPHFKCEKCNFKEDADYNAALNISNPKLKSTKEKP

SEQ ID NO: 1221 - protein, 726 aa, synthetic construct
SEVEFSHEYWMRHALTLAKRARDEREVPVGAILVLNNRVIGEGWNRTTGLHDPTAHAEIMALRQGGLVMQNYRLIDATLYVTFEPCVMCAGAMIHSRIGRVVFGVRNSKHGAAGSLVNVLNYPGMNHRVEITEGILVDECAALLCDFYRMPRRVFNAQKKAQSTINSGGSSGGSSGSETPGTSESPTPESSGGSPGGSAKNTITKTLKLRIVRPYNSAEVEKIVADEKNNREKIALEKNKDKVKEACSKHLKVASYCTTQVERNACPFCKARKLDDKFYQKLRGQFPDAVFWQELGEILRQLQKQAAEIYNQSLIELYYEIFIKGRGFANASIVEHYLSDVCYTRAAELFKNAAIASGLRGKVKSNFRLKELKNMKSGLPTTKSDNFPIPLVKQKGGQYTGFEISSHNDDFIIKIPFGRWQVKKEIDKYRPWEKFDFEQVRKSPKPISLLLSTQRRKRNKGWSKDEGTEAEIRKVMNGDYRTSYIEVKRGSKIGEKSAWMLNLSIDVPKIDKGVDPSIIGGIDVGVKSPLVCAINNAFSRYSISDNDLFHFNKKMFARRRILLKRNRHKRAGHGAKNKLKPITTLTEKSKRFRKKLIERWACEIADFFIKNKVGTVQMENLESMKRKEDSYFNIRLRGFWPYAEMQNKIEFKLRQYGIEIRKVAPNNTSKTCSKCGHLNNYFDFEYRRKNKFPLFKCEKCSFKENADYNAALNISNPKLKSTKGEP

SEQ ID NO: 1222 - protein, 726 aa, synthetic construct
SEVEFSHEYWMRHALTLAKRARDEREVPVGAVLVLNNRVIGVGWNRAIGLHDPTAHAEIMALRQGGLVMQNYRLIDATLYVTFEPCVMCAGAMIHSRIGRVVFGVRNSKRGAAGSLMNVLNYPGMNHRVEITEGVLADECAALLCDFYRMPRQVLNAQKKAQSSINSGGSSGGSSGSETPGASGSVIPKSSGGSSAGSTKDTITKTLKLRIVRPYNSAEVEKIVADEKNNREKIALEKNKDKVKEACSKHLKVAAYCTTQVERSACLFCKARRLDDKFYQKLRGQFPDAVFWQEIGEIFRQLQKQAAETYNQSLIELYYEIFIKGKGFANASSVEHYLSDVCYTRAAELFKNAAIASGLRGKVKSNFRLKELKNMKSGLPTTKSDNFPIPLVKQKGGQYTGFEISSHNDDFIIKIPFGRWQVKKEIDKYRPWEKFDFEQVRKSPKPISLLLSTRRRKRNKGWSKDEGTEAEIRKVMNGDYQTSYIEVKRGSKIGEKSAWMLNLSIDVPKIDKGVDPSIIGGIDVGVKSPLVCAINNAFSRYSISDNELFHFNKKMFARRRILLKKNRHKRAGHGAKNKLKPITILTEKSKRFRKKLIERWACEIADFFIKNKVGTVQMESLESMKRKEDSYFNIRLRGFWPYAEMQNKIEFKLKQYGIKIRKVAPNNTSKTCSMCGHLNNYFSFEYRKKNKFPHFKCEKCNFKENADYNAALNISNPKLKSTKEEP

SEQ ID NO: 1223 - protein, 726 aa, synthetic construct
SEVEFSHEYWMRHALTLAKRARDEREVPVGAVLVLNNRVIGEGWNRTTGLHDPTAHAEIMALRQGGLVMRNYRLTDATLYVTFEPCVMCAGAMIHSRIGRVVFGVRNSKRGAAGSLMNVLNYPGMNHCVEITEGILVDECAALLCDFYRMPRQVLNAQKKAQSSISPGGSSGGSSGSETPGASESVTPKSSGGSSGGSAKNTITKTLKLRIVRPYNSAEVEKIVADEKDNREKIALEKNKDKVKEACSKHLKVAAYCTTQVERNACLFCKARKLDDKFYQKLRGQFPDAVFWQEIGEIFRQLQRQAAEIYNQSLIELYYEIFIKGKGFANASSVEHYLSDVCYTRAAELFKNAAIASGLRGKVKSNFRLKELKNMKSGLPTTKSDNFPIPLVKQKGGQYTGFEISSHNDDFIIKIPFGGWQVKKEIDKYRPWEKFDFEQVRKSPKPISLLLSTQRRKRNKGWSKDEGTEAEIRKVMNGDYQTSYIEVKRGGKIGEKSAWMLSLSIDVPKVDKGVDPSIIGGIDVGVKSPLVCAINNAFSRYSISDNELFHFNKKMFARRRILLKKSRHRRAGHGAKNKLKPITILTEKSVRFRKKLIERWACEIADFFIKNKVGTVQMENLESMKRKEDSYFNIRLRGFWPYAEMQNKIEFKLKQYGVEIRRVAPNNTSRTCSKCGHLNNYFNFEYRRKNKFPHFKCEKCNFKEDADYNAALNISNPKLKSTREEP

SEQ ID NO: 1224 - protein, 726 aa, synthetic construct; identical to SEQ ID NO: 1128

SEQ ID NO: 1225 - protein, 726 aa, synthetic construct
SEVEFSHEYWMRHALTLAKRARDEREVPVGAVLVLNNRVIGEGWNRTTGLHDPTAHAEIMALRQGGLVMQNHRLVDATLYVTFEPCVMCAGAMVHSRIGRVVFGVRNSKRGAAGSLMNVLNYPGMNHCVEITEGILVDECAALLCDFYRMPRQVLNAQKKAQSSISSGGSSGGSGGSEPPGASESVTPKSSAGSSAGSTKSTITKTLKLRIVRPYNSAEVEKIVADEKNNREKIALEKNKDKVKEACSKHLKVAAYCTTQVERNACLFCKARKLDDKFYQKLRGQFPDAVFWQEIGEVFRQLQKQAAEIYNQSLIELYYEIFIKGKGFANASSVEHYLSDVCYARAAELFKNAAIASGLRGKVKSNFRLKELKNMRSGLPTTKSDNFPIPLVKQKGGQYTGFEISSHNDDFIIKIPFGRWQAKKEIDKYRPWEKFDFEQVRKSPKPISLLLSTQRRKRNKGWSKDEGTEAEIRKVMNGDYQTSYIEVKRGSKIGEKSAWMLNLSIDVPKIDKGVDPSIIGGIDVGVKSPLVCAINNAFSRYSISDNDLFRFNKKMFARRRILLRKNRHKRAGHGAKNKLKPITILTEKSVRFRKKLIERWACEIADFFIKNKVGTVQMENLESMKRKEDSYFNIRLRGFWPYAEMQNKIEFKLKQYGIEIRKVAPTNTSKTCSKCGHLNNYFNFEYRKKNKFPHFKCERCSFKENADYNAALNISNPKLRSTKEEP

SEQ ID NO: 1226 - protein, 726 aa, synthetic construct
SEVEFSHEYWMRHALTLAKRARDEREVPVGAVLVLNNRVIGEGWNRAIGLHDPTAHAEIMALRQGGLVMQNYRLIDATLYVTFEPCVMCAGAMVHSRIGRVIFGVRNSKRGAAGSLMNVLDYPGMGHRVEITEGILADECAALLCDFYCMPRQVFNAQKRAQSSINSGGSSGGSSGSETPGTSESATPESSGGSSGGSAKNTITKTLKLRIVRPYNSAEVEKIVADEKNNREKIALAKNKDKVKEACSEHLKVAAYCTTQVERNACLFCKARKLDDKFYQKLRGQFPDAVFWQEIGEVFRQLQKQAAEIYNQSLIELYYEIFIKGKGFANASSVEHYLSDVCYTRAAELFKNAAIASGLRGKVKSNFRLKELKNMKSGLPTTKSDNFPIPLVKQKGGQYTGFEISSHNDDFIIKIPFGRWQVKKEINKFRPWEKFDFEQVRKSPKPLSLLLSTQRRKRNKGWSRDEGTEAEIRKVMNGDYQTSYIEVKRGSKIGEKSAWMLNLSIDVPKIDKGVDPSIIGGIDVGVKSPLVCAINNAFSRYSISDNDLFHFNKKMFARRRILLKKTRHKRAGHGAKNKLKPISILTEKSERFRKKLIERWACEIADFFIKNKVGTVQMENLESMKRREDSYFNIRLRGFWPYAKMQNKIEFKLKQYGIEIRKVAPNNTSKTCSKCGHLNNYFNFEYRKKNKFPHFKCEKCNFKESADYNAALNISNPKLKSTKEEP

SEQ ID NO: 1227 - protein, 726 aa, synthetic construct
SEVEFSHEYWMRHALTLAKRARDEREVPVGAVLVLNNRVIGVGWNRAIGLHDPTAHAEIMALRQGGLVMQNYRLTDATLYVTFEPCVMCAGAMIHSRIGRVVFGVRNSKHGAAGSLMNVLNYPGMNHRVEITEGILADECAALLCDFYRMPRRVFNAQKKAQSSINSGGSSDGSSGSGTLGTSGSPTRESSGGGFGGSAKNTITKTLQLRIVRPYNSAEVEKIVADEKNNREKIALEKNKDKVKEACSKHLKVASYCTTQVERNACLFCKARKLDDKFYQKLRGQFPDAVFWQELGEIFRQLQKQAAEIYNQSLIELYYEIFIKGKGFANASSVEHYLSDVCYTRAAELFKNAAIASGLRGKVKSNFRLKELKNMKSGLPTTKSDNFPIPLVKQKGGQYTGFEISSHNDDFIIKVPFGRWQAKKEIDKYRPWEKFDFEQVRKSPKPISLLLSTQRRKRNKGWSKDEGTEAEIRRVMNGDYQTSYIEVKRGSKIGEKSAWMLNLSIDVPKIDKGVDPSIIGGIDVGVKSPLVCAINNAFSRYSISDNELFHFNKKMFARRRILLKKNRHKRAGHGVKNKLKPITILTEKSGRFRKKLIERWACEIADFFVKNKVGTVQMENLESMKRKEDSYFNIRLRGFWPYAEMQNKIEFKLKQYGIKVRKVAPNNTSKTCSKCGHLNNYFSFEYRKKNKFPHFKCEKCNFKENADYNAALNISNPKLKSTKEEP

SEQ ID NO: 1228 - protein, 726 aa, synthetic construct
SEVEFSHEYWMRHALTLAKRARDEREVPVGAVLVLNNRVIGEGWNRAIGLHDPTAHAEIMALRQGGLVTQNYRLIDATLYVTFEPCVMCAGAMVHSRIGRVVFGVRNSKRGAAGSLMNVLDYPGMGHRVEITEGILADECAALLCDFYCMPRQVFNAQKRAQSSINPGGSSGGSSGSETLGTSENATPESSGGSSGSSAKNTITKTLKLRIVRPYNSAEVEKIVADEKNSREKIALEKNKDKVKEACSKHLKVAAYCTTQVERNACLFCKARKLDDKFYQKLRGQFPDAVFWQEIGEIFRQLQKQAAETYNQSLIELYYEIFIKGKGIANASNVEHYLSDVCYTRAAELFKNAAIASGLRNKIKSNFRLKELRNMKSGLPTTKSDNFPIPLVRQKGGQYTGFEISNHNGDFIIKIPFGRWQVKKEIDRYRPWEKFDFEQVRKSPKPISLLLSTQRRKRNKGWSKDEGTEAEIRKVMNGDYRTSYIEVKRGSKIGEKGAWMLNLSIDVPKIDKGVDPSIIGGIDVGVKSPLVCAINNALSRYSISDNDLFHFNKKMFARRRILLRKNRHKRAGHGARNKLKPITVLTEKSERFRKKLIERWACEIANFFIKNKVGTVQMENLESMKRREDSYFNIRLRGFWPYAEMQNKIEFKLKQYGIEIRKVAPNNTSKTCSKCGHLNNYFNFEFRKKNKFPHFKCEKCNFKENADYNAALNISNPKLKSTKEEP

SEQ ID NO: 1229 - protein, 726 aa, synthetic construct
SEVEFSHEYWMRHALILAKRARDEREVPVGAVLVLNNRVIGVGWNRAIGLHDPTAHAEIMALRQGGLVMQNYRLSDATLYVTFEPCVMCAGAMIHSRIGRVVFGVRNSKRGAAGSLMNVLNYPGMNHCVEITEGILVDECAALLCDFYRMPRQVLSAQKKAQSSVSSGGSSGGSSGSETPGASGSVTPKSSVGSSASSTKNTITKTLKLRIVRPYNSAEVEKIVADEKNNREKIALEKNRDKVKEACSKHLKVAAYCTTQVERNACLFCKARKLDDKFYQKLRGQFPDAVFWQEIGEIFRQLQKQAAEIYNQSLVELYYEIFIKGKGIANASSVEHYLSDVCYTKAAELFKNAAIASGLRNKIKSNFRLKELRNMKSGLPTTKSDNFPIPLVRQKGGQYTGFEISNHNGDFIIKIPFGRWQVKKEISKHRPWEKFDFEQVRKSPKPISLLLSTQRRKRNKGWGKDEGTEAEIRKVMNGGYQTSYIEVKRGSKIGEKSAWMLSLSIDVPKIDKGVDPSIIGGIDVGVKSPLVCAINNALSRYSISDNDLFHFNKKMFARRRILLRKNRHKRAGHGARNKLKPITVLTEKSERFRKKLIERWACEIANFFIKNKVGTVQMENLESMKRREDSYFNIRLRGFWPYAEMQNRIELKLKQYGIEIRRVAPNNTSRTCSKCGHLNNYFNFEYRKKNKFPHFKCEKCNFREDADYNAALNISNPKLKSTKEEP

SEQ ID NO: 1230 - protein, 726 aa, synthetic construct
SEVEFSHEYWMRHALTLAKRARDEREVPVGAVLVLNNRVIGEGWNRAIGLHDPTAHAEIMALRQGGLVMQNYRLTDATLYVTFEPCVMCAGAMIHSRIGRVVFGVRNSKRGAAGSLMNVLNYPGMNHCVEITEGILMDECAALLCDFYRMPRQVLNAQKKAQSSISSGGPSGGSSCSETPGASGSVTPKSSVGSSAGSTKSTITKTLKLRIVRPYNSAEVEKIVADEKNNREKIALEKNKDKVKEACSKHLKVAAYCTTQVERNACLFCKARKLDDKFYQKLRGQFPDAVFWQEISEIFRQLQKQAAEIYNQSLIELYYEIFIKGKGFANASSVEHYLSDVCYTRAAELFKNAAIASGLRGKVKSNFRLKELKNMKSGLPTTKSDNFPIPLVKQKGGQYTGFEISSHHDDLIIKIPFGRWQVKKEIDKYRPWEKFDFEQVRKSPKPISLLLSTQRRKRNKGWSKDEGTEAEIRKVMNGDYQTSYIEVKRGSRIGEKSAWMLSLSIDVPKIDRGVDPSIIGGIDVGVKSPLVCAINNAFSRYSISDNDLFHFNKKMFARRRILLKKNRHRRAGHGAKNKLKPITILTEKSVRFRKKLIERWACEIADFFIKNKVGTVQMENLESMKRKEDSYFNIRLRGFWPYAEMQNKIEFKLKQYGIEIRKVAPNNTSKTCSKCGHLNSYFNFEYRKKNKFPHFKCEKCNFRENADYNAALNISNPKLRSTKEEP

SEQ ID NO: 1231 - protein, 726 aa, synthetic construct
SEVEFSHEYWMRHALTLAKRARDEREVPVGAILVLNNRVIGEGWNRAIGLHDPTAHAEIMALRQGGLVMQNYRLIDATLYVTFEPCVMCAGAMIHSRIGRVVFGVRNNKHGAAGSLVNVLNYPGMNHRVEITEGILADECAALLCDFYRMPRQVFNARKKAQSSINPGGSSGSSSGSETPGTSESATPESSGGSSGGSAKNTITKTLKLRIVRPYNSAEVEKIVADEKNNREKIALEKNKGKVKEACSKHLKVATYCTTQVGRNACLFCKARKLDDKFYQKLRGQFPDAVFWQEIGEIFRQLQKQAAEIYNQSLIELYYEILIKGKGIANASSVEHYLSDVCYTRAAELFKNAAIASGLRNKIKSNFRLKELRNMKSGLPTTKSDNFPIPLVKQKGGQYTGFEISSHNDDFIIKIPFGRWQMKKEIDKYRPWEKFDFEQVRKSPKPISLLLSTQRRKRNKGWSKDEGTEAEIRRVMNGDYQTSYIEVKRGSKIGEKSAWMLNLSIDVPKIDKGVDPSIIGGIDVGVRSPLVCAINNAFSRYSISDNDLFHFNKKMFARRRVLLKNNKHKRAGHGAKNKLKPISILTGKSERFRKKLIERWACEIADFFIRNKVGTVQMENLEGMKRKEDSYFNIRLRGFWPYAEMQNKIEFKLKQYGIEIRKVAPNNTSKTCSKCGHLNNYFNFGYRKRNKFPHFKCEKCNFKEDADYNAALNISNPKLKSTKEEP

SEQ ID NO: 1232 - protein, 726 aa, synthetic construct
SEVEFSHEYWMRHALTLAKRARDEREVPVGAVLVLNNRVIGEGWNRAIGLHDPTAHAEIMALRQGGLVMQNYRLSDATLYVTFEPCVMCAGAMIHSRIGRVVFGVRNSKRGAAGSLMNVLNYPGMNHCVEITEGILVDECAALLCDFYRMPRQILSAQKKAQSSISSGGSSGGSSGSETPGTSESVTPKSSGGSSAGSTKDAITKTLKLRIVRPYNSAEVEKIVADEKDSREKIALEKNRDKVKEACSKHLRLAAYCTTQVERNACLFCKARKLDDKFYRKLRGQFPDAVFWQELGEIFRQLQKQAAEIYNQSLIELYYEIFVKGKGIANTSRMEHYLSDVCYTRAAKLFKNAAIASGLRGKIKSNFRLKELKSMKSGLPTTRSDNFPIPLVKQKGGQYTGFEISSNDSDFIIKIPFGRWQVKKEIDKYRPWEKFDFEQVRKSPKPISLLLSTQRRKRNKGWSKDEGTEAEIKKVMNGDYQTSYIEVKRGSKIGEKSAWMLNLSIDVPKIDKGVDPSIIGGIDVGVKSPLVCAINNAFSRYSISDNDLFHFNKKMFARRRILLKKNRHKRAGHGVKNKLKPITILTEKSGRFRKKLIERWACEIADFFVKNKVGTVQMENLESMKRKEDSYFNIRLRGFWPYAEMQNKIEFKLKQYGIKVRKVAPNNTSKTCSKCGHLNNYFSFEYRKKNKFPHFKCEKCNFKENADYNAALNISNPKLKSTKEEP

SEQ ID NO: 1233 - protein, 726 aa, synthetic construct
SEVEFSHEYWMRHALTLAKRARDEREVPVGAVLVLNNRVIGEGWNRAIGLHDPTAHAEIMALRQGGLVMQNYRLTDATLYVTFEPCIMCAGAMIHSRIGRVVFGVRNSKRGAAGSLMNVLNYPGMNHRVEITEGILADECAALLCDYYRMPRQIFNARKKAQSSINSGGSSDGGSGSETPGTSESATPESSGGSSGGSAKNTITKTLKLRIVRPYNSAEVEKIVADEKNNREKIALEKNKDKVKEACSKHLKVAPYCTTQVERNACPFCKARKLDDKFYQKLRGQSPDAVFWQELGEIFRQLQKQAAEIYNQSLIELYYEIFIKGRGFANAGSVEHYLSDVCYTRAAELFKNAAIASGLRGKVKSNFRLKELKNMKSGLPTTKSDNFPIPLVKQKGGQYTGFEISSHNDDFIIKIPFGRWQVKKEIDKYRPWEKFDFEQVRKSPKPISLLLSTQRRKRNKGWSKDEGTEAEIRKVMNGDYQTSYIEVKRGSKTGEKSAWMLNLSIDVPKIDKGVDPSIIGGIDVGVKSPLVCAINNAFSRYSISDNDLFRFNKKVFARRRILLKKNRHKRAGHGAKNKLKPISILTGKSERFRKKLIERWACEIADFFIKNKVGTVQMENLESMKRKEDSYFNIRLRGFWPYAEMQNKIEFKLKQYGIEIRKVAPNNTSKTCSKCGHLNNYFNFEYRKKNKFPHFKCEKCNFKENADYNAALNISNPKLKSTKEKP

SEQ ID NO: 1234 - protein, 726 aa, synthetic construct
SEVEFSHEYWMRHALTLAERARDEREVPVGAILVLNNRVIGEGWNRAIGLHDPTAHAEIMALRQGGLVMQNYRLTDATLYVTFEPCVMCAGAMIHGRIGRVVFGARNSKRGAAGSLMNVLNYPGMNHCVEITEGILVDECAALLCDFYHMPRQVLNAQKKAQSSISSGGSSGGSSGSETPGASESVTPKSSGGSSAGSTKDTITKTLKLRIVRPYNSAEVEKIVADEKNSREKIALEKNKDKVKEACSEHLKVAAYCTTQVERNACLFCKARKLDDRFYQKLRGQFPDAVFWQETGEIFRQLQRQAAEIYNQSLIELYYEIFIKGKGFANASSVEHYLSDVCYTRAAELFKNAAIASGLRGKVKSNFRLKELKNMKSGLPTTKSDNFPIPLVKQKGGQYTGFEISSHNDDFIIKIPFGRWQVKKEIDKYRPWEKFDFEQVRKSPKPISLLLSTQRRKRNKGWGKDEGTEAEIRKVMNGDYQTSYIEVKRGSKIGEKSAWMLNLSIDVPRIDKGVDPSIIGGIDVGVKSPLVCAINNALSRYSISDNDLFHFNKKMFARRRILLRKNRHKRAGHGARNKLKPITVLTEKSERFRRKLIERWACEIANFFIKNKVGTVQMENLESMKRREDSYFNIRLRGFWPYAEMQSKIEFKLKQYGIKIRKVAPNNTSKTCSKCGHLNNYFNFEYRRKNKFPHFKCEKCNFKENADYNAALNISNPKLKSTKEEP

SEQ ID NO: 1235 - protein, 726 aa, synthetic construct
SEVEFSHEYWMRHALTLAKRARDEREVPVGAVLVLNNRAIGEGWNRAIGLHDPTAHAEIMALRQGGLVMQNYRLTDATLYVTFEPCVMCAGAMIHSRIGRVVFGVRNSKRGAAGSLMNVLNYPGMNHCVEITEGILMDECAALLCDFYRMPRQVLIAQKKAQSSISSGGSSGGSSCSVTPGTSESATPESSGGGFGGSAKNTITKTLQLRIVRPYNSAEVEKIVADEKNNREKIALEKNKDKVKEACSEHLKVAAYCTTQVERNACLFCKARKLDDRFYQKLRGQFPDAVFWQETGEIFRQLQKQAAEVYNQSLVELYYEILIKGKGIANASSVEHYLSDVCYTRAAELFKNAAIASGLRGKVKSNFRLKELKNMRSGLPTAKSDNFPIPLVKQKGGQYTGFEISSHNDDFIIKIPFGRWQVKKEIDKYRPWEKFDFEQVRKSPKPISLLLSTRRRKRNKGWSKDEGTEAEIRKVMNGDYQTSYIEVKRGSKIGEKSAWMLNLSIDVPKIDKGVDPSIIGGIDVGVKSPLVCAINNAFSRYSISDNDLFRFNKKMFARRRILLKKNRHKRAGHGAKNKLKPITILTGKSRRFRKKLIERWACEIADFFIKNKVGTVQMESLESMKRKEDSYFNIRLRGFWPYAEMQNKIEFKLKQYGIKIRKVAPNNTSKTCSKCGHLNNYFSFEYRKKNKFPHFKCEKCNFKENADYNAALNISNPKLMSTKEEP

SEQ ID NO: 1236 - protein, 726 aa, synthetic construct
SEVGFSHEYWMRHALTLAKRARDEREVPVGAVLVLNNRVIGEGWNRTTGLHDPTAHAEIMALRQGGLVTQNHRLVDATLYVTFEPCVMCAGAMIHSRIGRVVFGARNSKRGAAGSLMNVLSYPGMNHRVEITEGILADECAALICDYYRMPRQVFNARKKAQSSINSGGSSDGGSGSETPGTSESATPESSGGSSGGSAKNTITKTLKLRIVRPYNSAEVEKIVADEKNNREKIALEKNKDKVKEACSEHLKVAAYCTTQVERSACLFCKARKLDDKFYQKLRGQFPDAVFWQEIGEIFRQLQKQAAEIYNQSLIELYYEIFIKGKGFANASSVEHYLSDVCYTRAAELFKNAAIASGLRGKVKSNFRLKELKNMKSGLPTTKSDNFPIPLVKQKGGQYTGFEISSHNDDFIIKIPFGRWQVKKEIDKYRPWEKFDFEQVRKSPKPISLLLSTQRRKRNKGWGKDEGTEAEIKKVMNGDYQTSYIEVKRGSKIGEKSAWMLNLSIDVPKIDRGVDPSIIGGIDVGVKSPLVCAINNAFSRYSISDNDLFHFNKKVFARRRILLKNNRHRRAGHGAKNKLKPITILTEKSKRFRKKLIERWACEIADFFIKNKVGTVQMENLESMKRKEDSYFNIRLRGFWPYAEMQNKIEFKLKQYGIEIRKVAPNNTSKTCSKCGHLNNYFNFEYRKKNKFPHFKCEKCNFKENADYNAALNISNPKLKSTKEEP

SEQ ID NO: 1237 - protein, 726 aa, synthetic construct
SEDEFSHEYWMRHALTLAKRARDGREVPVGAVLVLNNRVIGEGWNRAIGLHDPTAHAEIMALRQGGLVMQNYRLIDATLYVTFEPCVMCAGAMVHSRIGRVVFGVRNSKRGAAGSLMNVLDYPGMDHRVEITEGILADECAALLCDFYRMPRQVFNAQKKAQSSINSGGSSGGSSGSETPSTSESATPESSGGSSGGSAKNTITKTLQLRIVRPYNSAEVEKIVTDEKNNREKIALEKNKDKVKEACSKHLKMASYCTTQVERNACLFCKARKLDDKFYQKLRGQFPDAVFWQELGEIFRQLQKQAAEIYNQSLIELYYEIFIKGKGFANASSVEHYLSDVCYTRAAELFKNAAIASGLRGKVKSNFRLKELKNMKSGLPTTKSDNFPIPLVKQKGGQYTGFEISSHNDDFIIKIPFGRWQVKKEVDKYRPWEKFDFEQVRKSPKPISLLLSTQRRKRNKGWSKDEGTEAEIRKVMNGDYQTSYIEVRRGSKIGERSAWMLNLSIDVPKIDKGVNPSIIGGIDVGVKSPLVCAINNAFSRYSISDNDLFRFNKKMFARRRILLKKNRHKRAGHGAKNKLKPITILTEKSGRFRKKLIERWACEIADFFVKNKVGTVQMENLESMKRKEDSYFNIRLRGFWPYAEMQNKIEFKLKQYGIKVRKVAPNNTSKTCSKCGHLNNYFSFEYRKKNKFPHFKCEKCDFKENADYNAALNISNPKLKSTKEEP

SEQ ID NO: 1238 - protein, 726 aa, synthetic construct
SEVEFSHEYWMRHALTLAKRARDEREVPVGAILVLNNRVIGEGWNRAIGLHDPTAHAEIMALRQGGLVMQNYRLIDATLYVTFEPCVMCAGAMIHSRIGRVVFGVRNSKHGAAGSLMNVLNYPGMNHRVEITEGILADECAALLCDFYRMPRQVFNARKKAQSSISPGGSSGGSSGSETPGTSESVTPESSGGSPGGSAKNTITKTLKLRIVRPYNSAEVEKIVVDEKNNREKIALEKNKDKVKEACSKHLEVAAYCTTQVERNACLFCKARKLDDKFYQKLRGQFPDAVFWQEIGEIFRQLQRQAAEIYNQSLIELYYEIFIKGKGFANASSVEHYLSDVCYTRAAELFKNAAIASGLRGKVKSNFRLKELKNMKSGLPTTKSDNFPIPLVKQKGGQYTGFEISSHNSDFIIKIPFGRWQVKEEIDKYRPWEKFDFEQVRKSPKPISLLLSTQRRKKNKGWSKDEGTEAEIRRVMNGDYQTSYIEVKRGSKIGEKSAWMLNLSIDVPKIDKGVDPSIIGGIDVGVKSPLVCAINNAFSRYSISDNDLFHFNKKMFARRRILLKKNRHKRAGHGAKNKLKPISILTEKSKRFRKKLIERWACEIADFFIKNKVGTVQMENLEGMKRKEDSYFNIRLRGFWPYAEMQNKIEFKLKQYGIKVRKVAPNNTSKTCSKCGHLNNYFSFEYRKKNKFPHFKCEKCNFRENADYNAALNISNPKLKSTKEEP

SEQ ID NO: 1239 - protein, 726 aa, synthetic construct
SEVEFSHEYWMRHALTLAKRARDEREVPVGAVLVLNNRVIGEGWNRAIGLHDPTAHAEIMALRQGGLAMRNYRLVDATLYVTFEPCVLCAGAMVHSRIGRVVFGVRNSKRGAAGSLMNVLNHPGMNHRVEITGGILADECAALLCDFYRMPRQVFNAQKKARSNINSGGSSGGSSGSETLGTSESATPESSGGSSGGSAKNTITKTLKLRIVRPYNSAEVEKIVADEKNNREKIALEKNKDKVKEACSEHLKVAAYCTTQVERNACLFCKARKLDDKFYQKLRGQFPDAVFWQEISEIFRQLQKQAAEIYNQSLIELYYEIFIKGKGFANASSVEHYLSDVCYTRAAELFKNAAIASGLRSKVKSNFRLKELKNMKSGLPTTKSDNFPIPLVKQKGGQYTGFEISSHNSDFIIKIPFGRWQVKEEIDKYRPWEKFDFEQVRKSPKPISLLLSTQRRKKNKGWSKDEGTEAEIRRVMNGDYRTSYIEVKRGSKIGEKSAWMLNLSIDVPKIDKGVDPSIIGGIDVGVKSPLVCAINNSSSRYSICDNDLFRFNKKMFARRRILLKKNRHKRAGHGAKNKLKPITILTKKSERFRKKLIERWACEVADFFIKNKVGTVQMENLESMKRKEDSYFNIRLRGFWPYAEMQNRIELKLKQYGIEIRRVAANNTSRTCSKCGHLNNYFNFEYRKKSKFPHFKCEKCNFREDADYNAALNISNPKLKSTKEEP

SEQ ID NO: 1240 - protein, 726 aa, synthetic construct
SEVESSHEYWMRHALALAKRARDEREVPVGAVLVLNNRVIGEGWNRAIGLHDPTAHAEIMALRQGGLVMQNYRLTDATLYVTFEPCVMCAGAMIHSRIGRVVFGVRNSKRGAAGSLMNVLNYPGMNHCVEITEGILVDECAALLCDFYRMPRQVLNAQKKAQSSISSGGSSGGSSGSETPGASGSVTPKSSGGSSACSTKDTITKTLKLRIVRPYNSAEVEKIVADEKNNREKIALEKNEDKVKEACSEHLKVAAYCTTQVERSACLFCKARKLDDKFYQKLRGQFPDAVFWQEIGEIFRQLQKQAAEIYNQSLIELYYEIFIKGKGFANASSVEHYLSDVCYTRAAELFKNAAIASGLRGKVKSNFRLKELKNMKSGLPTTKSDNFPIPLVKQKGGQYTGFEISSHNDDFIIKIPFGRWQVKKEIDKYRPWEKFDFEQVRKSPKPISLLLSTQRRKRNKGWSKDEGTEAEIKKVMNGDYQISYIEVKRGTKIGEKSAWMLNLSVDVPKIDKGVDPSIIGGIDVGVKSPLVCAINNALSRYSISDNDLFRFNKKMFARRRILLKKNRHKRAGHGAKNKLKPISILTEKSERFRKKLIEKWACEIADFFIKNKVGTVQMENLESIKRKEDSYFNIRLRGFWPYAEMQNKIEFKLKQYGIEIRKVAPNNTSKTCSKCGHLNNYFNFEYRKKNKFPHFKCEKCNFKENADYNAALNISNPKLKSTKEGP

SEQ ID NO: 1241 - protein, 726 aa, synthetic construct
SEVEFSHEYWMRHALTLAKRARDEREVPVGAVLVLNNRVIGEGWNRAVGLHDPTAHAEIMALHQGGLVMQNYRLIDATLYVTFEPCVMCAGAMIHSRIGRVVFGARNSKRGAAGSLMNVLSYPGMNHRVEITEGILADECAALLCDFYRMPRRVFNAQKKAQSSINSGGSSGGGSGSETPSTSESTTPESSGGSSGGPAKNTITKTLKLRIVRPYNSAEVEKIVADEKNNREKTALEKNKDKVKEACSKHLKVAAYCTTQVERNACLFCKARKLDDKFYQKLRGQFPDAVFWQELGEIFRQLQKQAAEIYNQSLIELYYEIFIKGKGFANASSVEHYLSDVCYTRAAELFKNAAIASGLRGKVKSNFRLKELKNMKSGLPTTKSDNFPIPLVKQKGGQYTGFEISSHNDDLIIKIPFGRWQVKREIDKYRPWEKFDFGQVRKSPKPISLLLSTQRRKRNRGWSKDEGTEAEIRKVMNGDYQTSYIEVKRGSKTGEKSAWMLNLSIDVPKIDKGVDPSIIGGIDVGVKSPLVCAINNAFSRYSISDNDLFRFNKKMFARRRILLKKNRHKRAGHGARNKLKPISILTEKSKRFRKKLIERWACEIADFFIKNKVGTVQMENLESMKRREDSYFNIRLRGFWPYAEMQNKIEFKLKQYGIVVRKVAPNNTSKTCSKCGHLNNYFNFEYRKKNKFPHFKCEKCNFKEDADYNAALNISNPKLKSTKGEP

SEQ ID NO: 1242 - protein, 726 aa, synthetic construct
SEVEFSHEYWMRHALTLAKRARDEREVPVGAVLVLNNRVIGEGWNRTTGLHDPTAHAEIMALRQGGLVMQNHRLVDATLYVTFEPCVLCAGAMVHSRIGRVVFGVRNSKRGAAGSLMNVLNHPGMNHRVEITGGILADECAALLCDFYRMPRQVFNAQKKARSNINSGGSSGGSSGSETLGTSESATPESSGGSSGGSAKNTIAKTLKLRIVRPYNSAEVEKIVADEKNNREKIALEKNKDKVKEACSKHLKVASYCTTQVERNACLFCKARKLDDKFYQKLRGQFPDAVFWQELGEIFRQLQKQAAEIYNQSLIELYYEIFIKGKGLANASSVEHYLSDVCYTRAAELFKNAAIASGLRGKVKSNFRLKELKNMKSGLPTTKSDNFPIPLVKQKGGQYTGFEVSSHNDDFIIKIPFGRWQVKKEIDKYRPWEKFDFEQVRKSPKPISLLLSTQRRKRNKGWSKDEGTEAEIRKVMNGDYQTSYIEVKRGSKIGEKSAWMLNLSIDVPKIDKGVDPSIIGGVDVGVKSPLVCAVNNAFSRYSISDNELFHFNKKMFARRRILLKKNRHKRAGHGAKNKLKPISTLTERSKRFRKKLIERWACEIADFFIKNKVGTVQMENLESMKRKEDSYFNIRLRGFWPYAEMQNKIEFKLRQYGIEIRKVASNNTSKTCSKCGHLNNYFNFEYRKKNKFPHFKCEKCNFKENADYNAALNISNPKLKSTKKEP

SEQ ID NO: 1243 - protein, 726 aa, synthetic construct
SEVEFSHEYWMRHALTLAKRARDEREVPVGAVLVLNNRVIGEGWNRAIGLHDPTAHAEIMALRQGGLVMQNYRLIDATLYVTFEPCVMCAGAMVHSRIGRVVFGVRNSKHGAAGSLVNVLNYPGMNHRIEITEGILADECAALLCDFYRMPRQVFNARKKAQSSINSGGSSGCSSGSEAPGASESVTPKSSGGSSGGSAKNTITKTLKLRIVRPYNSAEVEKIVADEKNNREKIALEKNEGKVKEACGKHLKVASYCTTQVERNACLFCKARKLDDKFYQKLRGQFPDAVFWQELGEIFRQLQKQAAEIYNQSLIELYYEIFIKGKGLANASSVEHYLSDVCYTRAAELFKNAAIASGLRGKVKSNFKLKELKSMKSGLPSTKSDNFPIPLVKQKGGQYTGFEISSYNDDLIIKIPFGRWQVKKEIDKYRPWEKFDFEQVRKSPKPISLLLSTQRRKRSKGWSKDEGTEAEIRKVMNGDYQTSYIEVKRGSKIGEKSAWMLNLSIDVPKIDKGVDPSIIGGIDVGVKSPLVCAINNAFSRYSISDNDLFRFNKKMFARRRILLKKNRHKRAGHGAKNKLKPISILTERSERFRKKLIERWACEIADFFIKNKVGTVQMENLESMKRKEDSYFNIRLRGFWPYAEMQNKIEFKLKQYGIEIRKVAPNNTSKTCSKCGHLNNYFNFEYRKKNKFPHFKCEKCNFKEDADYNAALNISNPKLKSTKEEP

SEQ ID NO: 1244 - protein, 726 aa, synthetic construct
SEVEFSHEYWMRHALTRAKRARDEREVPVGAILVLNNRVIGEGWNRAIGLHDPTAHAEIMALRQGGLVMQNYRLIDATLYVTFEPCVMCAGAMIHSRIGRVVFGVRNSKRGAAGSLMNVLDYPGMGHRVEITEGILADECAALLCDFYCMPRQVFNAQKRAQSSINSGGSSGGSSGSETPGTSESATPESSGGGSSGSAKNTITKTLQLRIVRPYNSAEVEKIVADEKSNREKIALEKNKDKVREACSKHLKVASYCTTQVERNACPFCKARKLDDKFYQKLRGQFPDAVFWQEIGEIFRQLQKQAAEIYNQSLIELYYEIFIKGKGFANASRVEHYLSDVCYTRAAELFKNAAIASGLRGKVKSNFKLKELKSMKSGLPSTKSDNFPIPLVKQKGGQYTGFEISSHNDDFIIKIPFGRWQVKKEIDKYRPWEKFDFEQVRKSPKPISLLLSTQRRKRNKGWSKDEGTEAEIRRVMNGDYQTSYIEVKRGSKIGEKSAWVLNLSIDVPKIDKGVDPSIIGGIDVGVRSPLVCAINNAFSRYSISDNDLFRFNKKMFARRRILLKKNRHKRAGHGAKNKLKPITILTEKSRRFRKKLIERWAREIADFFIKNKVGTVQMESLESMKRKEDSYFNIRLRGFWPYAEMQNKIEYKLKQYGIKVRKVAPNNTSKTCSKCGHLNNYFSFEYRKKNKFPHFKCEKCNFKENADYNAALNISNPKLKSTKEEP

SEQ ID NO: 1245 - protein, 726 aa, synthetic construct
SEVEFSHEYWMRHALTLAKRARDEREVPVGAILVLNNRVIGEGWNRAIGLHDPTAHAEIMALRQGGLVMQNYRLIDATLYVTFEPCVMCAGAMIHSRIGRVVFGVRNSKHGAAGSLVNVLNYPGMNHRVEITEGILADECAALLCDFYRMPRQVFNARKKAQSSINPSGSSGGSSGSVTPGTSESATPESSGGGFGGSAKNTITKTLQLRIVRPYNSAEVEKIVADEKNNREKIALEKNKDKVKEACSKHLKVASYCTTQVERNACLFCKARKLDDKFYQKLRGQFPDAVFWQELGEIFRQLQKQAAEIYNQSLIELYYEIFIKGKGIANASSVEHYLSDVCYTRAAELFKNAAIASGLRNKIKSNFRLKELKNMKSGLPTTKSDNFPIPLVKQKGGQYTGFEISSHNDDFIIKIPFGRWQVKKEIDKYRPWEKFDFEQVRKSPKPISLLLSTQRRKRNKGWSKDEGTEAEIRKVMNGDYQTSYIEVKRGSKIGEKSAWMLNLSIDVPKIDKGVDPGIIGGIDVGVKSPLVCAINNAFSRYSIGDNDLFHYNKKMFARRRILLKKNRHKRAGHGAKNKLKPISILTEKSKRFRKKLIERWACEIADFFIKNKVGTVQIENLESMKRKEDSYFNIRLRGFWPYAEMQNKIEFKLKQYGIEIRKVAPNNTSKTCSKCGHLNSYFNFEYRRKYKFPHFKCEKCNFKEDADYNAALNISNPKLKSTKEEP

SEQ ID NO: 1246 - protein, 726 aa, synthetic construct
SEVEFSHEYWMRHALTLAKRARDEREVPVGAILVLNNRVIGEGWNRAIGLHDPTAHAEIMALRQGGLVMQNYRLIDATLYVTFEPCVMCAGAMIHSRIGRVVFGVRNSKHGAAGSLVNVLNYPGMNHRVEITEGILADECAALLCDFYRMPRQVFNARKKALSSTNSGGSSDGGSGSETPGTSESATPESSGGSSGGSAKNTITKTLKLRIVRPYNSAEVEKIVADEKSNREKIALEKNKDKVKEACSKHLKVAAYCTTQVERNACLFCKARKLDDKFYQKLRGQFPDAVFWQEIGEVFRQLQKQAAEIYNQSLIELYYEIFIKGKGYANASSVEHYLSDVCYTRAAGLFKNAAIASGLRGKVKSNFKLKELKSMKSGLPSTKSDNFPIPLVKQRGGQYTGFEISSHNDDFIIKIPFGRWQAKKEIDKYRPWEKFDFEQVRKSPKPISLLLSTQRRKRNRGWSKDEGTEAEIRKVMNGDYQTSYIEVKRGSKFGEKSAWMLNLSIDVPKIDKGVDPSIIGGIDVGVKSPLVCAINNAFSRYSISDNDLFRFNKKMFARRRILLGKNRHKRAGHGVKNKLKPITILTEKSGRFRKKLIERWACEIADFFVKNKVGTVQMENLESMKRKEDSYFNIRLRGFWPYAEMQNKIEFKLKQYGIKVRKVAPNNTSKTCSKCGHLNNYFSFEYRKKNKFPHFKCEKCNFKENADYNAALNISNPKLKSTKEEP

SEQ ID NO: 1247 - protein, 726 aa, synthetic construct
SEVEFSHEYWMRHALTLAKRARDEREVPVGAVLVLNNRVIGVGWNRAIGLHDPTAHAEIMALRQGGLVMQNYRLTDATLYVTFEPCVMCAGAMVHSRIGRVVFGVRNSKRGAAGSLMNVLNYPGMSHCVEITEGILVDECAALLCDFYRMPRQVLNAQKKAQSSISSGGSSGGSGGGETPGASESVTPKSSGGSSAGSTKNTITKTLKLRIVRPYNSAEVEKIVADEKNSREKIALEKNRDRVKEACSEHLKVAAYCTTQVERSACLFCKARKLDDRFYQKLRGQFPDAVFWQEISEIFRQLQKQAAEIYNQSLIELYYEIFIKGKGFANASSVEHYLSDVCYTRAAELFKNAAIASGLRGKVKSNFRLKELKNMKSGLPTTKSDNFPIPLVKQKGGQYTGFEISSHNSDFIIKIPFGRWQVKEEIDKYRPWEKFDFEQVRKSPKPISLLLSTQRRKKNKGWSKDEGTEAEIRRVMNGDYQTSYIEVKRGSKIGEKSAWMLNLSIDVPRIDKGVDPSIIGGIDVGVKSPLVCAINNAFGRYSISDNDLFHFNKKMFARRRILLKKNRHKRAGHGAKNKLKPITILTEKSKRFRKKLIERWACEIADFFIKNKVGTVQMENLESMKRKEDSYFNIRLRGFWPYAEMQNKIEFKLKQYGIEIRKVAPNNTSRTCSKCGHLNNYFSFEYRKKNKFPHFKCEKCNFKEDADYNAALNISNPKLKSTKEEL

SEQ ID NO: 1248 - protein, 726 aa, synthetic construct
SEVEFSHEYWMRHALSLAKRARDEREVPVGAVLVLNNRIIGEGWNRAIGQHDPTAHAEIMALRQGGLVMQNNRLTDATLYVTFEPCVMCAGAMVHSRIGRVVFGVRNSKRGAAGSLMNVLNYPGVNHCVEITEGILVDECAALLCDFYRMPRQVLNAQKKAQSSISSGGSSGGCSGSEMPGASESVTPKSSGGGSAGSTKNTITKTLKLRIVRPYNSAEVEKIVADEKNSREKIALERNKDKVKEACSEHLKVAAYCTTQVERNACLFCKARKLDDRFYQKLRGQFPDAVFWQETGEIFRQLQRQAAEIYNQSLIELYYEIFIKGKGFANASSVEHYLSDVCYTRAAELFKNAAIASGLRGKVKSNFRLKELKNMKSGLPTTKSDNFPIPLVKQKGGQYTGFEISNHNGDFVIKIPFGRWQVKKEINKHRPWERFDFEQVRKSPKPISLLLSTQRRKRNKGWSKDEGTEAEIRKVMNGDYQTSYIEVKRGSKIGEKSAWMLNLSIDVPKIDKGVDPSITGGIDVGVKSPLVCAINNAFSRYSISDNDLFHFNKKMFARRRILLKKNRHKRAGHGAKNKLKPITILTEKSGRFRKKLIERWACEIADFFIKNKVGTVQMENLGSMKRKEDSYFNIRLRGFWPYAEMQNKIELKLKQYGIKIRKVAPNNTSKTCSKCGHLNDYFNFEYRKKNKFPHFKCEKCNFKEDADYNAALNISNPKLKGTREEP

SEQ ID NO: 1249 - protein, 726 aa, synthetic construct
SEVEFSHEYWMRHALTLAKRARDEREVPVGAVLVLNNRVIGEGWNRAIGLHDPTAHAEIMALRQGGLVMQNYRLIDATLYVTFEPCVMCAGAMIHSRIGRVVFGVRNNKRGAAGSLMNVLNYPGMNHRVEITEGILADECAALLCDFYRMPRQVLNAQKKARSCINPGGSSGGSSGSETPGTSESATPESSGGGSSGSAKNTITKTLQLRIVRPYNSAEVEKIVADEKNNRERIALEKNKDKVREACSKHLKVASYCTTQVERNACPFCKARKLDDKFYQKLRGQFPDAVFWQELGEILRQLQKQAAEIYNQSLIELYYEIFIKGRGFANASSVEHYLSDVCYTRAAELFKNAAIASGLRGKVKSNFRLKELKNMKSGLPTTKSDNFPIPLVRQKGGQYTGFEISNHDGDFIIKIPFGRWQVKKETDKYRPWEKFDFEQVRKSPKPISLLLSTQRRKRNRGWSKDESTEAEIKKVMNGDYQTSYIEVKRGSKTGEKSAWMLNLSIDVPKIDKGVDPSIIGGIDVGVKSPLVCAINNALSRYSISDNDLFRFNKKMFARRRILLKKNRHKRAGHGAKNKLKPISILTGKSERFRKKLIERWACEIADFFIKNKVGTVQMENLESMKRKEDSYFNIRLRGFWPYAEMQNKIEFKLKQYGIEIRKVAPNNTSKTCSKCGHLNNYFNFEYRKKNKFPHFKCEKCNFKESADYNAALNISNPKLKSTKGEP

SEQ ID NO: 1250 - protein, 726 aa, synthetic construct
SEVEFSHEYWMRHALTLAKRARDEREVPVGAVLVLNNRVIGEGWNRAIGLHDPTAHAEIMALRQGGLVMQNYRLSDATLYVTFEPCVMCAGAMIHSRIGRVVFGVRNSKRGAAGSLMNVLNYPGMNHCVEITEGILVDECAALLCDFYRMPRQVLSAQKKAQSSISSGGSSGGSSGSETPGASGSVTPKSSVGSSAGSTQNTITKTLKLRIVRPYNSAEVEKIVADEKNNREKIALEKNKDKVKEACSKHLKVASYCTTQVERNACPFCKARKLDDKFYQKLRGQFPDAVFWQELGEIFRQLQKQAAEIYNQSLIELYYEIFIKGKGIANASRVGHYLSDVCYTRAAELFKNAAIASGLRNKIKSNFRLKELKNMKSGLPTTKSDNFPIPLVKQKGGQYTGFEISNHNSDFIIKIPFGRWQVKKEIDRYRPWEKFDFEQVRKSPKPISLLLSTQRRKRNKGWGKDEGTEAEIRKVMNGDYQTSYIEVKRGSKIGEKSAWMLNLSIDVPKIDKGVDPSIIGGIDVGVKSPLVCAINNALSRYSISDNDLFHFNKKMFARRRILLRKNRHKRAGHGARNKLKPITVLTEKSERFRKKLIERWACEIANFFIKNKVGTVQMENLESMKRREDSYFNIRLRGFWPYAEMQNKIEFKLKQYGIKIRKVAPNNTSKTCCKCGHLNNYFNFEFRKKNKFPHFKCEKCNFKEDADYNAALNISNPKLKSTKEEP

SEQ ID NO: 1251 - protein, 726 aa, synthetic construct
SEVEFSHEYWMRHALTLAKRARDEREVPVGAVLVLNNRVIGEGWNRAIGLHDPTAHAEIMALRQGGLVMQNYRLIDATLYVTFEPCVMCAGAMIHSRIGRVVFGVRNSKHGAAGSLVNVLNYPGMNHRVEITEGILADECAALLCDFYRMPRQVFNARKKAQSSINPGGSSGGSSGSETQGTSESATPESSGGSSGGSAKNTITKTLKLRIVRPYNSAEVEKVVADEKNNREKIALEKNKDKVKEACSKHLKVAAYCTTQVERNACLFCKARKLDDGFYQKLRGQFPDAVFWQEIGEIFRQLQKQAAEIYNQSLIELYYEIFIKGKGFANASSVEHYLSDVCYTRAAELFKNAAIASGLRNKTKSNFRLKELRSMKSGLPTTKSDNFPIPLVKQKGGQYTGFEISNHNSDFIIKIPFGRWQAKKEIDKYRPWEKFDFEQVRKSPKPISLLLSTQRRKRNKGWSKDEGTEAEIRKVMNGDYQTSYIEVKRGSRIGEKSAWMLSLSIDVPKIDRGVDPSIIGGIDVGVKSPLVCAINNALSRYSISDNDLFHFNKKMFARRRILLKKNRHKRAGHGAKNKLKPISILTEKSKRFRKKLIERWACEIADFFIKNKVGTVQMENLEGMKRKEDSYFNIRLRGFWPYAEMQNKIEFKLKQYGIEIRKVAPNNTSKTCSKCGHLNNYFNFEYRKKNKFPHFKCEKCNFKENADYNAALNISNPKLKSTREEP

SEQ ID NO: 1252 - protein, 726 aa, synthetic construct
SEVEFSHEYWMRHALTLAKRARDEREVPVGAILVLNNRVIGEGWNRAIGLHDPTAHAEIMALRQGGLVMQNYRLTDATLYVTFEPCVMCAGAMVHSRIGRVVFGVRNNKRGAAGSLMNVLDYPGMDHRVEITEGILADECAALLCDFYRMPRQVFNAQRKAQSSINSGGSSGGSSGSETPGTSESATPESSGGSSGGSAKNTITKTLQLRIVRPYNSAEVEKIVADEKNSREKIALEKNKDKVKEACSKHLMVASYCTTQVERSACLFCKARELDGKFYQKLRGQFPDAVFWQELGEIFRQLQKQAAEIYNQSLIELYYEIFVKGKGIANASSVEHYLSDVCYTRAAELFKNAAIASGLRNKVKSNFRLKELRNMKSGLPTTKSDNFPIPMVKQKGGQYTGFEISSHNDDFIIKIPFGRWQVKKEIDKYRPWEKFDFEQVRKSPKPISLLLSTQRRRRNKGWSKDEGTEAEIRKVMNGDYQTSYIEVKRGSKIGEKSAWMLSLSIDVPKIDKGVDPSIIGGIDVGVKSPLVCAINNAFCRYSISDNDLFHFNKKMFARRRILLKKSRHKRAGHGAKNKLKPISILTEKSKRFRKKLIERWACEIADFFIKNKVGTVQMENLESMKRKEDSYFNIRLRGFWPYAEMQNKIEFKLKQYGIVVRKVAPNNTSKTCSKCGHLNNYFNFEYRKKNKFPHFKCEKCNFKESADYNAALNISNPKLKSTKEEP

SEQ ID NO: 1253 - protein, 726 aa, synthetic construct
SEVEFSHEYWMRHALTLAKRARDEREVPVGAVLVLNNRVIGEGWNRAIGLQDPTAHAEIMALRQGGLVMQNYRLSDATLYVTFEPCVMCAGAMIHSRIGRVVFGVRNSKRGAAGSLMNVLNYPGMNHCVEITEGILVDECAALLCDFYRMPRQVLSAQKKAQSSVSSGGSSGGSSGSETPGASGSVTPKSSVGSSAGSTKNTITKTLKLRIVRPYNSAEVEKIVADEKNNREKIALEKNRDKVKEACSKHLKVAAYCTTQVERNACLFCKARKLDDKFYQKLRGQFPDAVFWQELGGIFRQLQKQAAEIYNQSLVELYYEILIKGKGIANASSVEHYLSDVCYTRAAELFKNAAIASGLRNKIKSNFRLKELRNMKSGLPTTKSDNFPIPLVRQKGGQYTGFEISNHDGDFIIKIPFGRWQVKKEINKHRPWEKFDFEQVRKSPKPISLLLSTQRRKRNKGWSKDEGTEAEIRKVMNGDYQTSYIEVKRGSKTGEKSAWMLNLSIDVPKIDKGVDPSVVGGIDVGVKSPLVCAINNAFSRYSISDNDLFHFNKKMFARRRILLKKNRHKRAGHGAKNKLKPISILTEKSERFRKKLIERWACEIADFFIRNKVGTVQMENLESMKRKEDSYFNIRLRGFWPYAEMQNKIEFKLKQYGIKIRKVAPNNTSRTCSECGHLNNYFSFEYRKKNKFPHFKCEKCNFKEDADYNAALNISNPKLKSTKEEP

SEQ ID NO: 1254 - protein, 726 aa, synthetic construct
SEVEFSHEYWMRRALTLAKRARDEREVPVGAVLVLNNRVIGVGWNRAVGLHDPTAHAEIMALRQGGLVMQNYRLIDATLYVTFEPCIMCAGAMIHSRIGRVVFGVRNSKRGAAGSLMNVLNYPGMNHRVEITEGILADECAALLCDFYRMPCQVFNARKKAQSSISPGGPSGGSSGSETPGTSESAAPESPGGSSGGSAKNTITKTLKLRIVRPYNSAEVEKIVADEKNSREKIALEKNKDKVKEACSEHLKVAAYCTTQVERNACLFCKARKLDDGFYQKLRGQFPDAVFWQETGEIFRQLQRQAAEIYNQSLIELYYEIFIKGKGFANASSVEHYLSDVCYTRAAELFKNAAIASGLRGKVKSNFRLKELKNMKSGLPTTKSDNFPIPLVKQKGGQYTGFEISSHNHDFIIKIPFGRWQVKKEIDKYRPWEKFDFEQVRKSPKPISLLLSTQRRRRNKGWSRDEGTEAEIRKVMNGDYQTSYIEVKRGSKIGEKSAWMLSLSIDVPKIDKGVDPSIIGGIDVGVKSPLVCAINNAFCRYSISDNDLFHFNKKMFARRRILLKKSKHKRAGHGAKNKLKPITILTEKSRRFRKKLIERWACEIADFFIKNKVGTVLMENLESMKRKEDSYFNIRLRGFWPYAEMQNKIEFKLKQYGIEVRKVAPNNTSKTCSKCGHLNNYFNFEYRKKNKFPHFKCEKCNFKENADYNAALNISNPKLKSTKEEP

SEQ ID NO: 1255 - protein, 726 aa, synthetic construct
SEVEFSHEYWMRHALALAKRARDEREVPVGAVLVLNNRAIGEGWNRAIGLHDPTAHAEIMALRQGGLVMQNYRLTDATLYVTFEPCVMCAGAMIHSRIGRVVFGVRNSKRGAAGSLMNVLNYPGMNHCVEITEGILVDECAALLCDFYRMPRQVLNTQKKAQSSISSGGSSGGSSGSETPGASGSVTPKSSGGSSAGSTKDTITKTLKLRIVRPYNSAEVEKVVADEKNNREKIAIEKNKDMVKEACSKHLKVASYCTTQVERNACLFCKARKLDDKFYQKLRGQFPDAVFWQELGEIFRQLQKQAAEIYNQSLIELYYEIFIKGKGLANASSVEHYLSDVCYTRAAELFKNAAIASGLRGKVKSNFKLKELKSMKSGLPSTKSDNFPIPLVKQRGGQYTGFEISSHNDDFIIKIPFGKWQAKKEIDKYRPWEKFDFEQVRKSPRPISLLLSTQRRKRNKGWSKDEGTEAEIKKVMNGDYQTSYIEVKRGSKIGEKSAWMLSLSIDVPKIDKGVDPSIIGGIDVGVKSPLVCAINNAFSRYSISDNDLFHFNKKMFARRRILLKKNRHKRAGHGAKNKLKPISILTEKSKRFRKKLIERWACEIADFFIKNKVGTVQMENLESMKRKEDSYFNIRLRGFWPYAEMQNKIEFKLKQYGIEIRKVAPNNTSKTCSKCGHLNNYFNFEYRKMNKFPHFKCEKCNFKENADYNAALNISNPKLKSTKEEP

SEQ ID NO: 1256 - protein, 726 aa, synthetic construct; identical to SEQ ID NO: 684

SEQ ID NO: 1257 - protein, 726 aa, synthetic construct
SEVEFSHEYWMRHALTLAKRARDEREVPVGAILVLNNRVIGEGWNRAIGLHDPTAHAEIMALRQGGLVMQNYRLTDATLYATFEPCVMCAGAMIHSRIGRVVFGVRNSKHGAAGSLMNALNYPGMNHRVEITEGILADECAGLLCDFYRMPRQVFSARKKAQSSINPGGSSGGSSGGKAPGTSESATLESSGGSSGGSAKNSITKTLKLRIVRPYNSAEVEKIVADEKNNREKTALEKNKGKVKEACSKHLKVATYCTTQVERNACLFCKARKLDDKFYQKLRGQFPDAVFWQEIGEIFRQLQKQAAEIYNQSLIELYYEIFIEGKGSANARSVEHYLSDVCYTRAAELFKNAAIASGLRGKVKSNFRLKELKNMKSGLPTTKSDNFPIPLVKQKGGQYTGFEVSSHNDDFIIKIPFGRWQEKKEINKYRPWEKFDFAQVRKSPKPISLLLSTQRRKRNRGWSKDESTEAEIRKVMNGDYQTSYIEVKRGSKIGEKSAWMLNLSIDVPKIDKGVDPSIIGGIDVGVKSPLVCAINNAFSRYSISDNDLFHFNKKMFARRRILLKKSKHKRAGHGAKNKLKPITILTEKSKRFRKKLIERWACEIADFFIKNKVGTVQMENLESMKKKEDSYFNIRLRGFWPYAEMQNKIEFKLKQYGIEIRKVAPNNTSRTCSKCGHLNNYFNFEYRKKNKFPHFKCEKCNFKEDADYNAALNISNPKLKSTKEEP

SEQ ID NO: 1258 - protein, 726 aa, synthetic construct
SEVEFSHEYWMRHALTLAKRARDEREVPVGAVLVLNNRVIGEGWNRAIGLHDPTAHAEIMALRQGGLVMQNYRLTDATLYVTFEPCVMCAGAMIHSRIGRVVFGVRNSKRGAAGSLMNVLNYPGMNHCVEITEGILVDECAALLCDFYRMPRQVLSAQKKAQSSISPGGSSGGSSGSETPGASESATPESSGGSSGGSAKNTITKTLKLRIVRPYNSAEVEKIVADEKNSREKIALEKNKDKVKEACSKHLKVAAYCTTQVERNACLFCKARKLDDKFYQKLRGQFPDAVFWQEIGEVFRQLQKQAAEIYNQSLIELYYEIFIKGKGFANASSVEHYLSDVCYTRAAELFKNAAIASGLRGKVKSNFRLKELKNMKSGLPTTKSDNFPIPLVKQKGGQYTGFEISSHNDDFIIKIPFGRWQVKKEINKFRPWEKFDLEQVRKSPKPISLLLSTQRRKRNKGWSKDEGTEAEIRKVMNGDYQTSYIEVKRGSKTGEKSAWMLNLSINVPKIDKGVDPSIIGGIDVGVKSPLVCAINNAFSRYSISDNDLFRFNKKMFARRRILLKKNRHKRAGHGAKNKLKPITILTEKSKRFRRKLIERWACEIADFFIKNKVGTVQMENLESMKRKEDSYFNIRLRGFWPYAEMQDKIEFKLKQYGIEIRKVAPNNTSKTCSRCGHLNNYFNFEYRRKSKFPHFKCEKCNFKENADYNAALNISNPKLKSTKEEP

SEQ ID NO: 1259 - protein, 726 aa, synthetic construct
SEVEFSHEYWMRHALTLAKRARDEREVPVGAVLVLNNRVIGEGWNRAVGLHDPTAHAEIMALRQGGLVMQNYRLVDATLYVTFEPCVLCAGAMVHSRIGRVVFGVRNSKRGAAGSLMNVLDYPGMNHRVEITEGILADECAALLCDFYRMPRQVFNARKKAQSSISPGGSSGGSSGSETPGASGSVTPKSSGGSSAGSTKDTITKTLKLRIVRPYNSAEVEKIVADEKNSREKIALEKNKDKVKEACSEHLKVAAYCTTQVERDACLFCKARKLDDKFYQKLRGQFPDAVFWQEIGEIFRQLQKQAAEIYNQSLIELYYEIFIKGKGFANASSVEHYLSDVCYTRAAELFKNAAIASGLRGKVKSNFRLKELKNMKSGLPTTKSDNFPIPLVRQKGGQYTGFEISSHNDDFIIKIPFGRWQVKEEIDKYRPWEKFDFEQVRRNPKPISLLLSTQRRKRNRGWSKDEGTEAEIRKVMNGDYQTSYVEVKRGSKIGEKSAWMLNLSIDVPKIDKGVDPSIIGGIDVGVKSPLVCAINNAFSRYSIGDNDLFRFNKKMFARRRILLGKNRHKRAGHGVKNKLKPITILTEKSGRFRKKLIERWACEIADFFVKNKVGTVQMENLESMKRKEDSYFNIRLRGFWPYAEMQNKIEFKLKQYGIKVRKVAPNNTSKTCSKCGHLNNYFSFEYRKKNKFPHFKCEKCNFKENADYNAALNISNPKLKSTKEEP

SEQ ID NO: 1260 - protein, 726 aa, synthetic construct
SEVEFSHEYWMRHALTLAKRARDEREVPVGAVLVLNNRVIGEGWNRTTGLHDPTAHAEIMALRQGGLVMQNHRLVDATLYVTFEPCVMCAGAMIHSRIGRVVFGVRNSKRGAAGSLTNVLNYPGMNHRVEITEGILVDECAALLCDFYRMPRQVFNAQKKAQSTINSGGSSGGSSGSETPGTSESPTPESSGGSPGGSAKNTITKTLKLRIVRPYNSAEVEKIVADEKNNREKIALEKNKDKVKEACSKHLKVAAYCTTQVERNACLFCKARKLDDKFYQKLRGQFPDAVFWQEIGEIFRQLQKQAAEIYNQSLIELYYEIFIKGKGFANASSVEHYLSDVCYTRAAELFKNAAIASGLRGKVKSNFRLKELKNMKSGLPTTKSDNFPIPLVKQKGGQYTGFEISSHNDDFIIKIPFGRWQVKKEIDKYRPWEKFDFEQVRKSPKPISLLLSTQRRKRNKGWSKDEGTEAEIRKVMNGDYQTSYIEVKRGSKTGEKSAWMLNLSIDVPKIDKGVDPSIIGGIDVGVKSPLVCAINNAFSRYSISDNDLFHFNKKMFARRRILLKKTRHKRAGHGAKNKLKPISILTEKSERFRKKLIERWACEIADFFVKNKVGTVQMENLESMKRKEDSYFNIRLRGFWPYAEMQNKIEFKLKQYGIKVRKVAPNNTSKTCSKCGHLNNYFSFEYRKKNKFPHFKCEKCNFKENADYNAALNISNPKLKSTKEEP

SEQ ID NO: 1261 - protein, 726 aa, synthetic construct
SEVEFSHEYWMRHALTLAKRARDEREVPVGAILVLNNRVIGEGWNRAIGLHDPTAHAEIMALRQGGLVMQNYRLIDATLYVTFEPCVMCAGAMIHSRIGRVVFGVRNSKHGAAGSLVNVLNYPGMNHRVEITEGILADECAALLCDFYRMPRQVFGARRKAQSSINPGGSSGGSSGSETPGTSESPTPESPGGSSGGSAKNTITKTLQLRIVRPYNSAEVEKIVADEKNNREKIALEKNKDKVKEACSKHLKVASYCTTQVERNACLFCKARKLDDKFYQKLRGQFPHAVFWQELGEIFRQLQKQAAEIYNQSLIELYYEIFIKGKGFANASSVEHYLSDVCYTRAAELFKNAAIASGLRGKVKSNFRLKELKSMKSGLPTTKSDNFPIPLVKQKGGQYTGFEISSHNDDFIIKIPFGRWQVKKEIDKYRPWEKFDFEQVRKNPKPISLLLSTQRRKRNKGWSKDEGTEAEIRKVMNGDYQTSYIEVKRGSKIGEKSAWMLNLSIDVPKIDKGVDPSIIGGIDVGVKSPLVCAINDAFSRYSISDNDLFRFNKKVFARRRILLKKNRHKRAGHGTKNKLKPITILTEKSGRFRKKLIERWACEIANFFIKNKVGTVQMENLESMKRREDSYFNIRLRGFWPYAEMQNKIEFKLKQYGIEIRKVAPNNTSKTCSKCGHLNNYFNFEYRKKNKFPHFKCEKCSFKENADYNAALNISNPKLKSTKEEP

SEQ ID NO: 1262 - protein, 726 aa, synthetic construct
SEVEFSHEYWMRHALTLAKRARDEREVPVGAVLVLNNRVIGEGWNRAIGLHDPTAHAEIMALRQGGLVMQNYRLIDATLYVTFEPCVMCAGAMVHSRIGRVVFGVRNSKRGAAGSLMNVLDYPGMDHRVEITEGILADECAALLCDFYRMPHQVFNAQKKAQSSINSGGSSDGSSGSVTPGLSESATPESSGGSSGSSAKNTITKTLKLRIVRPYNSAEVEKIVADEKNNREKIALEKNKDKVKEACSKHLKVAAYCTTQVERNACLFCKARKLDDKFYQKLRGQFPDAVFWQEIGEIFRQLQKQAAEIYNQSLIELYYEIFIKGKGFANASSVEHYLSDVCYTRAAELFKNAAIASGLRGKVKSNFRLKELKNMKSGLPTTKSDNFPIPLVKQKGGQYTGFEISSHNDDFIIKIPFGRWQAKKEIDKYRPWEKFDFGQVRKSPKPISLLLSTQRRKRNKGWSKDEGTEAEIRKVMNGDYQTSYIEVKRGSKIGEKSAWMLSLSIDVPKIDKGVDPSIVGGIDVGVKSPLVCAINNAFNRYSISDNNLFHFNKKMFARRRILLKKNRHKRAGHGAKNKLKPISILTEKSERFRKKLIERWACEIADFFVRNKVGTVQMENLEGMKRKEDSYFNIRLRGFWPYAEMQNKIEFKLKQYGIEVRKVAPNNTSRTCSKCGHLNNYFNFEYRKKNKFPHFKCEKCNFKENADYNAALNISDPKLKSTKEEP

SEQ ID NO: 1263 - protein, 726 aa, synthetic construct
SEDEFSHEYWMRHALTLAKRARDGREVPVGAVLVLNNRVIGEGWNRAIGLHDPTAHAEIMALRQGGLVMQNYRLIDATLYVTFEPCVMCAGAMVHSRIGRVVFGVRNSKRGAAGSLMNVLDYPGMGHRVEITEGILADECAALLCDFYCMPRQVFNAQKRAQSSINSGSSSGGSSGSETPGTSESATPESSGGGFGGSAKNTITKTLQLRIVRPYNSAEVEKIVADEKNNREKIALEKNKDKVKEACSEHLKVAAYCTTQVERSACLFCKARKLDDKFYQKLRGQFPDAVFWQEIGEIFRQLQKQAAEIYNQSLIELYYEIFIKGKGFANASSVEHYLSDVCYARAAELFKNAAIASGLRGKVKSNFRLKELKNMRSGLPTTKSDNFPIPLVKQKGGQYTGFEISSHNDDFIIKIPFGRWQVKKEIDKYRPWEKFDFEQVRKSPKPISLLLSTQRRKRNKGWSKDEGTEAEIRKVLNGDYQTSYIEVKRGSKTGEKSAWMLNLSINVPKIDKGVDPSIIGGIDVGVKSPLVCAINNAFSRYSISDNDLFRFNKKMFARRRILLKKNRHKRAGHGAKNKLKPISILTGKSERFRKKLIERWACEIADFFIKNKVGTVQMENLESMKRKEDSYFNIRLRGFWPYAEMQNKIEFKLKQYGIEIRKVVPNNTSKTCSKCGHLNNYFNFEYRKKNKFPHFKCEKCNFKENADYNAALNISNPKLKSTKEKP

SEQ ID NO: 1264 - protein, 726 aa, synthetic construct
SEVEFSHEYWMRHALTLAKRARDEREVPVGAVLVLNNRVIGEGWNRAIGLYDPTAHAEIMALRQGGLVMQNYRLIDATLYVTFEPCVMCAGAMIHSRIGRVVFGVRNNKHGAAGSLVNVLDYPGMNHRVEITEGILADECAALLCDFYRMPRQVFNARKKAQSSISPGGSSGGSSGSETPGTSESATPESSGGSSGGSAKNTITKTLKLRIVRPYNSAEVEKIVADEKNNREKIALEKNKGKVKEACSKHLKVAAYCTTQVERNACLFCRARKLDDKFYQKLRGQFPDAVFWQEIGEVFRQLQKQAAEIYNQSLVELYYEIFIRGKGIANASSVEHYLSDVCYTRAAELFKNAAIASGLRGKVKSNFRLKELKSMKSGLPTTKSDNFPIPLVKQKGGQYTGFEISSHNDDFIIKIPFGRWQVKKEIDKYRPWEKFDFEQVRKSPKPISLLLSTQRRKRNKGWSKDEGTEAEIRKVMNGDYQTSYIEVKRGSKIGEKSAWMLNLSIDVPKIDKGVDPSIIGGIDVGVKSPLVCAINNALSRYSISDNDLFHFNKKMFARRRILLKKNRHRRAGHGAKNKLKPLTILTGKSKRFRKKLIERWACEIAGFFIKNKVGTVQLENLESMKRREDSYFNIRLRGFWPYAEMQNKIEFKLKQYGIEIRKVAPNNTSKTCSRCGHLNNYFNFEYRKRNKFPHFKCEKCNFKENADYNAALNISNPKLKSPKEEP

SEQ ID NO: 1265 - protein, 726 aa, synthetic construct
SEVEFSHEYWMRRALTLAKRARDEREVPVGAVLVLNNRVIGVGWNRAVGLHDPTAHAEIMALRQGGLVMQNYRLVEATLYVTFEPCIMCAGAMIHSRIGRVVFGVRNSKRGAAGSLMNVLNYPGMNHRVEITEGILADECAALLCDYYRMPRQVFNARKRAQSSINSGGSSDGGSGSETPGTSESATPESSGGSSAGPTKNTITKTLKLRIVRPYNSAEVEKIVADEKNSREKIALERNKDKVKEACSEHLKVAAYCTTQVERNACLFCKARKLDDRFYQKLRGQFPDAVFWQELGEILRQLQKQAAEIYNQSLIELYYEIFIKGRGFANASSVEHYLSDVCYTRAAELFKNAAIASGLRGKVKSNFRLKELKNMKSGLPTTKSDNFPIPLVRQKGGQYTGFEISNHDGDFIIKIPFGRWQVKEEINKHRPWEKFDFEQVRKSPKPISLLLSTQRRKRNKGWSKDEGTEAEIRKVMNGDYQTSYIEVKRGSKIGEKSAWMLNLSIDVPKIDKGVDPSIIGGIDVGVKSPLVCAINNALSRYSISDNDLFHFNKKMFARRRILLRKNRHKRAGHGAKNKLKPITMMTEKSKRFRKKLIERWAREIADFFIKNKVGTVQMENLESMKRKEDSYFNIRLRGFWPYAEMQDKIEFKLKQYGIVVRKVAPNNTSKTCSKCGHLNHYFNFEYRKKNKFPHFKCEKCNFKEDADYNAALNISNPKLKSTKGEP

SEQ ID NO: 1266 - protein, 726 aa, synthetic construct
SEVEFSHEYWMRHALTLARRARDGREVPVGAVLVLNNRVIGEGWNRAIGLHDPTAHAEIMALRQGGLVMQNYRLIDATLYVTFEPCVMCAGAMVHSRIGRVVFGVRNSKRGAAGSLMNVLDYPGMGHRVEITEGILADECAALLCDFYCMPRQVFSAQKRARPSINSGGSSGGSSGSDTPGISESATPESSGGGSSGSAKNTITKTLQLRIVRPYNSAEVEKIVADEKNNREKIALEKNKDKVREACSKHLKAASYCTTQVERNACPFCKARKLDDKFYQKLRGQFPDAVFWQELGGIFRQLQKQAAEIYNQSLIELYYEIFIKGKGFANASSVEHYLSDVCYTRAAELFKNAAIASGLRGKVKSNFRLKELKNMKSGLPTTKSDNFPIPLVKQKGGQYTGFEISSHNDDFIIKIPFGRWQVKKEIDKYRPWEKFDFEQVRKSPKPISLLLSTQRRKRNKGWSKDEGTEAEIRKVMNGDYQTSYIEVKRGSKIGEKSAWMLSLSIDVPKIDKGVDPSIIGGIDVGVKSPLVCAINNAFCRYSISDNDLFHFNKKMFARRRILLKKSRHRRAGHGAKNKLKPISILTEKSKRFRKKLIERWACEIADFFIKNKVGTVQMENLESMKRKEDSYFNIRLRGFWPYAEMQNKIEFKLKQYGIEIRKVAPNNTSKTCSKCGHLNSYFNFEYRKKNKFPHFKCEKCNFKENADYNAALNISNPKLKSTKEEP

SEQ ID NO: 1267 - protein, 726 aa, synthetic construct
SEGEFSHEYWMRHALTLAKRARDGREVPVGAVLVLNNRVIGEGWNRAIGLHDPTAHAEIMALRQGGLVMQNYRLIDATLYVTFEPCVMCAGAMIHSRIGRVVFGVRNNKHGAAGSLVNVLNYPGMNHRVEITEGILADECAALLCDFYRMPRQVFNARKKAQSSINPGGSSGGSSGSETPGTSESATPESSGGSSGSSAKNTITKTLKLRIVRPYNSAEVEKIVADEKNNREKIALEKNKDKVKEACSKHLKVAAYCTTQVERNACLFCKARRLDDKFYQKLRGQFPDAVFWQEIGEIFRQLQKQAAEVYNQSLVELYYEILIKGKGIANASSVEHYLSDVCYTRAAELFKNAAIASGLRNKIKSNFRLKELRNMKSGLPTTKSDNFPIPLVRQKGGQYTGFEISNHDGDFIIKIPFGRWQVKKEIDKYRPWEKFDFEQVRKSPKPISLLLSTQRRKRNKGWSKDVGTEAEIRKVMNGDYQTSYIEVKRGSKIGEKSAWMLNLSIDVPKIDKGVDPSIIGGIDVGVKSPLVCAINSAFSRYSISDNDLFRFNKRMFARRRILLKKNRHRRAGHGAKNKLKPITILTEKSRRFRKKLIERWACEIADFFIKNKVGTVQMESLESMKRKEDSYFNTRLRGFWPYAEMQNKIEFKLKQYGIKIRKVAPNNTSKTCSKCGHLNNYFNFEFRKKNKFPHFKCEKCNFKEDADYNAALNISNPKLKSTKEEP

SEQ ID NO: 1268 - protein, 726 aa, synthetic construct
SEVEFSHEYWMRHALTLAKRARDEREVPVGAVLVLNNRVIGEGWNRAIGLHDPTAHAEIMALRQGGLVMQNYRLADATLYVTFEPCVMCAGAMIHSRIGRVVFGVRNSKHGAAGSLVNVLNYPGMNHRVEITEGILADECAALLCDFYRMPRQVFNARKKAQPSINPSGSSGGSSGSVTPGTSESATPESSGGGFGGSAKNTITKTLQLRIVRPYNSAEVEKIVADEKNNREKIALEKNKDKVKEACSKHLKVASYCTTQVERNACLFCKARKLDDKFYQKLRGQFPDAVFWQELGEIFRQLQKQAAEIYNQSLIELYYEIFIKGKGLANASSVEHYLSDVCYTRAAELFKNAAIASGLRGKVKSNFKLKELKSMKSGLPSTKSDNFPIPLVKQRGGQYTGFEIGSHNDDFIIKIPFGRWQAKKEIDKYRPWEKFDFEQVRKSPKPISLLLSTQRRKRNKGWSKDEGTEAEIRKVMNGDYQTSYIEVKRGRKIGERSAWMLNLSIDVPKIDKGVDPNTIGGIDVGVKSPLVCAINNAFSRYSISDNDLFRFNKKMFARRRILLKKNRHKRAGHGAKNKLKPITILTEKSGRFRKKLIERWACEIADFFIKNKVGTVQMENLESMKRKEDSYFNIRLRGFWPYAEMQNKIELKLKQYGIKIRKVAPNNTSKTCSRCGHLNDYFNFEYRKKNKFPHFKCEKCNLKEDADYNAALNISNPKLKSTKEEP

SEQ ID NO: 1269 - protein, 726 aa, synthetic construct
SEVEFSHEYWMRHALTLAKRARDGREVPVGAVLVLNNRVIGEGWNRAIGLHDPTAHAEIMALRQGGLVMQNYRLIDATLYVTFEPCVMCAGAMVHSRIGRVVFGVRNSKRGAAGSLMNVLDYPGMGHRVEITEGILADECAALLCDFYCMPRQVFNAQKRAQSSINSGGPSGGSSGSETPGTSESATPESSGGGSSGSAKNTITKTLQLRIVRPYNSAEVEKIVADEKNNREKIALEKNKDKVKEACSKHLKVASYCTTQVERNACPFCKARKLDDKFYQKLRGQFPDAVFWQELGEILRQLQKQAAEIYNQSLIELYYEIFIKGRGFANASSVEHYLSDVCYTRAAELFKNAAIASGLRGKVKSNFRLKELKNMKSGLPTTKSDNFPIPLVKQKGGQYTGFEISSHNDDFIIKIPFGRWQVKKEIDKYRPWEKFDFEQVRKSPKPISLLLSTQRRKRNRGWSKDEGTEAEIRKVMNGDYQTSYIEVKRGSKTGEKSAWMLNLSIDVPKIDKGVDPSIIGGIDVGVKSPLVCAINNAFSRYSISDNDLFRFNKKMFARRRILLKKNRHKRAGHGAKNKLKPISILTGKSERFRKKLIERWACEIADFFIKNKVGTVQMENLESMKRKEDSYFNIRLRGFWPYAEMQNKIEFKLKQYGIEIRKVAPNNTSKTCSKCGHLNNYFNFEYRKKNKFPHFKCEKCNFKENADYNAALNISNPKLKSTKEEP

SEQ ID NO: 1270 - protein, 726 aa, synthetic construct
SEVEFSHEYWMRRALTLAKRARDEREVPVGAVLVLNNRVIGVGWNRAVGLYDPTAHAEIMALRQGGLVMQNYRLIEATLYVTFEPCIMCAGAMIHSRIGRVVFGVRNSKRGAAGSLMNVLNYPGMNHRVEITEGILADECAALLCDYYRMPRQVFNARKKVQSSINSGGSSDGGSSSETPGTSESATPESSGGSSGGSAKNTITKTLKLRIVRPYNSAEVEKIVADEKNNREKIALEKNKDKVKEACSEHLKVAAYCTTQVERSACLFCKARKLDDKFYQKLRSQFPDAVFWQEIGEIFRQLQKQAAEIYNQSLIELYYEIFIKGKGIANASSVEHYLSDVCYTRAAELFKNAAIASGLRNKIKSNFRLKELRNMKSGLPTTKSDNFPIPLVRQKGGQYTGFEISNHNGDFIIKIPFGRWQVKKEISKHRPWEKFDFEQVRKSPKPISLLLSTQRRKRNKGWGKDEGTEAEIRKVMNGDYQTSYIEVKRGSKIGEKSAWMLNLSIDVPKIDKGVDPSIIGGIDVGVKSPLVCAINNALSRYSISDNDLFHFNKKMFARRRILLRKNRHKRAGHGARNKLKPITVLTEKSERFRKKLIERWACEIANFFIKNKVGTVQMENLESMKRRGDSYFNIRLRGFWPYAEMQSKIEFKLKQYGIKIRKVAPNNTSKTCSKCGHLNNYFNFEFRKKNKFPHFKCEKCNFKEDADYNAALNISNPKLKSTKEEP

SEQ ID NO: 1271 - protein, 726 aa, synthetic construct
SEVEFSHEYWMRHALTLAKRARDGREVPVGAVLVLNNRVIGEGWNRAIGLHDPTAHAEIMALRQGGLVMQNYRLIDATLYVTFEPCVMCAGAMIHSRIGRVVFGVRNNKHGAAGSLVNVLNYPGMNHRVEITEGILADECAALLCDFYRMPRQVFNARKKAQSSINPGGSSGGSSGSETPGTSESATPESSGGSSGSSAKNTITKTLKLRIVRPYNSAEVEKIVADEKNNREKIALEKNKDKVKEACSKHLKVAAYCTTQVERNACLFCKARKLDDKFYQKLRGQFPDAVFWQEIGEIFRQLQKQAAEIYNQSLIELYYEIFIKGKGFANASSVEHYLSDVCYTRAAELFKNAAIASGLRGKVKSNFRLKELKNMKSGLPTTKSDNFPIPLVKQKGGQYTGFEISSHNDDFIIKIPFGRWRVKKEIDKYRPWEKFDFEQVRKSPKPISLLLSTQRRKRNKGWSKDEGTEAEIRKVMNGDYQTSYIEVKRGSKIGEKSAWMLNLSIDVPKIDKGVDPSIIGGIDVGVKSPLVCAINNALSRYSISDNDLFHFNKKMFARRRILLKKNRHRRAGHGARNKLKPITVLTEKSERFRKKLIERWACEIANFFVKNKVGTVQMENLESMKRKEDSYFNIRLRGFWPYAEMQNKIEFKLKQYGIEIRKVTPNNTSKTCSKCGHLNNYFSFEYRKKNKFPHFKCEKCNFKENADYNAALNISNPKLMSTKEGP

SEQ ID NO: 1272 - protein, 726 aa, synthetic construct
SEVEFSHEYWMRHALTLAKRARDEREVPVGAVLVLNNRVIGEGWNRAIGLHDPTAHAEIMALRQGGLAMQNYRLVDATLYVTFEPCVLCAGAMVHSRIGRVVFGVRNSKRGAAGSLMNVLNHPGMNHRVEITGGILADECAALLCDFYRMPRQVFNAQKKAQSSINSGGSSGGSSGSETPSTSESATPESSGGSSGGSAKNTITKTLQLRIVRPYNSAEVEKIVADEKNNREKIALEKNKDKVKEACSEHLKVAAYCTTQVERNACLFCKARKLDDKFYQKLRGQFPDAVFWQELGGIFRQLQKQAAEIYNQSLIELYYEIFIKGKGITNASRVEHYLSDVCYTRAAELFKNAAIASGLRGKVKSNFRLKELKNMKSGLPTTKSDNFPIPLVKQKGGQYTGFEISSHNDDFIIKIPFGRWQGKKEVDKYRPWEKFDFEQVRKGPKPISLLLSTQRRKRNRGWSKDEGTEAEIRKVMNGDYQTSYIEVKRGSKIGEKSAWMLNLSIDVPKIDMGVDPSIIGGIDVGVKSPLVCAINNAFSRYSISDNDLFHFNKKMFARRRILLKKNRHKRAGHGAKNKLKPISILTEKSKRFRKKLIERWACEIADFFIKNKVGTVQMENLESMKRKEDSYFNIRLRGLWPYAEMQNKIEFKLKQYGIKIRKVAPNNTSKTCSKCGHLNNYFNFEYRRKNKFPHFKCEKCNFKEDADYNAALNISNPKLKSTKEEP

SEQ ID NO: 1273 - protein, 726 aa, synthetic construct
SEVEFSHEYWMRHALTLAKRARDEREVPVGAVLVLNNRVIGEGWNRTAGLHDPTAHAEIMALRQGGLVMQNHRLVDATLYVTFEPCVMCAGAMIHSRIGRVVFGVRNSKRGAAGSLTNVLNYPGMNHRVEITEGILVDECAALLCDFYRMPRQVFNAQKKAQSTINSGGSSGGSSGSGTPGTSESPTPESSGGSSGGSAKNTITKTLKLRIVRPYNSTEVEKIVADEKNNREKIALEKNKDKVKEACSKHLKVASYCTTQVERNACLFCKARKLDDKFYQKLRGQFPDAVFWQELGEIFRQLQKQAAEIYNQSLIELYYEIFIKGKGFANASSVEHYLSDVCYTRAAELFKNAAIASGLRGKVKSNFRLKELKNMKSGLPTTKSDNFPIPLVKQKGGQYTGFEISSHNDDFIIKIPFGRWQVKKEIDKYRPWEKFDFEQVRKSPKPISLLLSTQRRKRNKGWSKDEGTEAEIRKVMNGDYQTSYIEVKRGSKIGEKSAWMLNLSIDVPKIDKGVDPSIIGGIDVGVKSPLVCAINNAFSRYSIIDNDLFHYNKKMFARRRILLKKNRHKRAGHGAKNKLKPTSILTEKSKRFRKKLIERWACEIADFFIKNKVGTVQIENLESMKRKEDSYFNIRLRGFWPYAEMQNKIEFKLKQYGIEIRKVAPNNTSKTCSKCGHLNSYFNFEYRKKNKFPHFKCEKCNFRENADYNAALNISNPKLRSTKEEP

SEQ ID NO: 1274 - protein, 726 aa, synthetic construct
SEVEFSHEHWMRHALTLAKRARDEREVPVGAVLVLNNRVIGEGWNRAIGLHDPTAHAEIMALRQGGLVLQNYRLVDATLYVTFEPCVLCAGAMVHSRIGRVVFGARNSKRGAAGSLMNILNYPGMNHRVEITEGILADECAALLCDFYRMPRQVFNAQKKAQSSINSGGSSSGSSGSETPGTSESATPESSGGGSSGSAKNTITKTLQLRIVRPYNSAEVEKIVADEKSNREKIALEKNKDKVREACSKHLKVASYCTTQVERNACPFCKARKLDDKFYQKLRGQFPDAVFWQELGEILRQLQKQAAEIYNQSLIELYYEIFIKGKGIASASRVGHYLSDVCYTRAAELFKNAAIASGLRGKVKSNFRLKELKNMKSGLPTTKSDNFPIPLVKQKGGQYTGFEISSHNSDFIIKIPFGRWQVKEEIDKYRPWEKFDFEQVRKSPKPISLLLSTQRRKKNKGWSKDEGTEAEIRRVMNGDYQTSYIEVKRGSKIGGKSAWMLNLSIDVPKIDKGVDPSIIGGIDVGVKSPLVCAINNSFSRYSICDNDLFRFNKKMFARRRILLKKNRHKRAGHGAKNKLRPITILTKKSERFRKKLIERWVCEVADFFIKNKVGTVQMENLESMKRKEDSYFNIRLRGFWPYAEMQNKIEFKLKQYGIEIRRVAPNNTSRTCSKCGHLNNYFNFEYRRKNKFPHFKCEKCNFKEDADYNAALNISNPKQKSTKEEP

SEQ ID NO: 1275 - protein, 726 aa, synthetic construct
SEVEFSHEYWMRHALTLAKRARDEREVPVGAVLVLNNRVIGEGWNRAIGLHDPTAHAEIMALRQGGLVMQNYRLIDATLYVTFEPCVMCAGAMIHSRIGRVVFGVRNSKHGAAGSLVNVLSYPGMNHRVEVTEGILADECAALLCDFYRMPRQVFGARRKAQSSINPGGSSGGSSGSETPGTSESPTPESSGGSSGGSAKNTITKTLQLRIVRPYNSAEVEKIVADEKNNREKIALEKNKDKVKEACSKHLKVASYCTTQVERNACPFCKARKLDDKFYQKLRGQFPDAVFWQELGEILRQLQKQAAEIYNRSLIELYYEIFIKGRGFANASSVEHYLSDVCYTRAAELFKNAAIASGLRGKVKSNFRLKELKNMKSGLPTTKSDNFPIPLVKQKGGQYTGFEISRHNDDFIIKIPFGRWQVKKGIDKYRPWEKFDFEQVRKSPKPISLLLSTQRRKRNKGWSKDEGTEAEIRKVMNGDYQTSYIEVKRGSKTGEKSTWMLNLSIDVPKIDKGVDPSIIGGIDVGVKSPLVCAINNAFSRYSISDNDLFRFNKKMFARRRILLKKNRYKRAGHGAKNKLRPISILTGKSERFRKKLIERWACEIADFFIKNKVGTVQMENLESMKRKEDSYFNIRLRGFWPYAEMQNKIEFKLKQYGIEIRKVAPNNTSKTCSKCGHLNNYFNFEYRRKNKFPHFKCEKCNFKEDADYNAALNISNPKLKSTKEEP

SEQ ID NO: 1276 - protein, 726 aa, synthetic construct
SEVEFSHEYWMRHALTLAKRARDEREVPVGAVLVLDNRVIGEGWNRAIGLHDPTAHAEIMALRQGGLVMQNYRLINATLYVTFEPCVMCAGAMIHSRIGRVVFGVRNSKHGAAGSLMNVLNYPGMNHRVEITEGILADECAALLCDFYRMPRQVFSARKKAQSSINSGGSSGGNSGNKTPGTSESATPEGSGGSSGGSVKNTITKTLKLRIVRPYNSAEVEKIVADEKNNREKIALEKNKDKVKEACSKHLKVASYCTTQVERNACLFCKARKLDDKFYQKLRGQFPDAVFWQELGGIFRQLQKQAAEIYNQSLIELYYEIFIKGKGITNASRVEHYLSDVCYTRAAELFKNAAIASGLRGKVKSNFRLKELKNMKSGLPTTKSDNFPIPLVKQKGGQYTGFEISSHNDDFIIKIPFGRWQVKREIDKYRPWEKFDFEQVRKSPRPISLLLSTQRRKRNKGWSKDEGTEAEIRKVMNGDYQTSYIEVKRGSKIGEKSAWMLNLSIDVPKIDKGVDPSIIGGIDVGVKSPLVCAINNAFSRYSISDNDLFHFNKKMFARRRILLKKTRHKRAGHGAKNKLKPISILTEKSERFRKKLIERWACEIADFFIKNKVGTVQMENLESMKRREDSYFSTRLRGFWPYAKMQNKIEFKLKQYGIEIRKVAPNNTSKTCSKCGHLNNYFNFEYRKKNKFPHFKCEKCNFKENADYNAALNISNPKLKSTKEEP

SEQ ID NO: 1277 - protein, 726 aa, synthetic construct
SEDEFSHEYWMRHALTLAKRARDEREVPVGAVLVLNNRVIGEGWNRTTGLHDPTAHAEIMALRQGGLVMRNYRLTDATLYVTFEPCVMCAGAMIHSRIGRVVFGVRNSKRGAAGSLMNVLNYPGMNHCVEITEGILVDECAALLCDFYRMPRQVFNARKKAQSSINPGGSSGGSGGSETPGTSESATPENSGGSSGSSAKNTITKTLKLRIVRPYNSAEVEKIVADEKNNREKIALEKNKDKVKEACSRHLKVAAYCTTQVERNACLFCKARRLDDKFYQKLRGQFPDAVFWQEIGEIFRQLQKQAAEIYNQSLVELYYEILIKGKGIANASSVEHYLSDVCYTRAAELFKNAAIASGLRNKVKSNFRLKELRNMKSGLPTTKSDNFPIPLVKQKGGQYTGFEISNHNSDFIIKIPFGRWQAKKEIDKYRPWEKFDFEQVRKSPKPISLLLSTQRRKRNRGWSKDEGTEAEIRRVMNGDYRTSYIEVKRGSKIGEKSAWMLNLSIDVPKIDKGVDPSIIGGIDVGVKSPLVCAINNAFSRYSISDNDLFHYNKKMFARRRILLKKNRHKRAGHGAKNKLKPISTLTGKSERFRKKLIERWACEIADFFIKNKVGTVQMENLESMKRKEDSYFNIRLRGFWPYAEMQNKIEFKLKQYGIEIRKVAPNNTSKTCSKCGHLNNYFNFEYRKKNKFPHFKCEKCNFKENADYNAALNISNPKLKSTKEEP

SEQ ID NO: 1278 - protein, 726 aa, synthetic construct
SEVEFSHEYWMRHALTLAKRARDEREVPVGAVLVLDNRVIGEGWNRAIGLHDPTAHAEIMALRQGGLAMQNYRLVDATLYVTFEPCAMCAGAMVHSRIGRVVFGVRNSKRGAAGSLMNVLNYPGMDHRVEITGGILADECAALLCDFYRMPRRVFNAQKKAQSSINSGGSSGGSSGSVTPGTSESATPESSGGSTGGSAKSTITKTLRLRIVRPYNSAEVEKIVADEKNNREKIALEKNKDKVKEACSKHLKVAAYCTTQVERNACLFCKARKLDDKFYQKLRGQFPDAVFWQEIGEIFRQLQKQAAEIYNQSLVELYYEIFIKGKGIANASSVEHYLSDVCYTRAAELFKNAAIASGLRNKIKSNFRLKELRNMKSGLPTTKSDNFPIPLVRQKGGQYTGFEISNHNGDFIIKIPFGRWQVKKEISKHRPWEKFDFEQVRKSPKPISLLLSTQRRKRNKGWGKDEGTEAEIRKVMNGDYQTSYIEVKRGSKIGEKSAWMLNLSIDVPKIDKGVDPSIIGGIDVGVKSPLVCAINNALSRYSISDNDLFHFNKKMFARRRILLRKNRHKRAGHGARNKLKPITVLTEKSERFRKKLIERWACEIANFFIKNKVGTVQMENLESMKRREDSYFNIRLRGFWPYAEMQSKIEFKLKQYGIEIRKVAPNNTSKTCSKCGHLNNYFNFEYRKRNKFPHFKCEKCNFKENADYNAALNISNPKLKSTKEKP

SEQ ID NO: 1279 - protein, 726 aa, synthetic construct; identical to SEQ ID NO: 684

SEQ ID NO: 1280 - protein, 726 aa, synthetic construct
SEVEFSHEYWMRHALTLAKRARDEREVPVGAILVLNNRVIGEGWNRAIGLNDPTAHAEIMALRQGGLVMQNYRLIDATLYVTFEPCVMCAGAMIHSRIGRVVFGVRNSKRGAAGSLMNVLNYPGMNHCVKITEGILVDECAALLCDFYRMPRQVLSAQKKAQSSISSGGSSGGCSGSEMPGASESVTPKSSGGSSAGSTKNTITKTLKLRIVRPYNSAEVEKIVADEKNSREKIALERNKDKVKEACSEHLKVAAYCTTQVERNACLFCKARKLDDKFYQKLRGQFPDAVFWQEIGEIFRQLQKQAAEIYNQSLIELYYEIFIKGKGFANASSVEHYLSDVCYTRAAELFKNAAIASGLRSKVRSNFRLKELKNMKSGLPTTKSDNFPIPLVKQKGGQYTGFEISSHNSDFIIKIPFGRWQEKEEIDKYRPWEKFDFEQVRKSPKPISLLLSTQRRKKNKGWSKDEGTEAEIRRVMNGDYQTSYIEVKRGSKIGEKSAWMLNLSIDVPKIDKGVDPSIIGGIDVGVKSPLVCAINNAFSRYSISDNDLFHFNKKMFARRRILLKKNRHRRAGHGAKNKLKPITILTEKSVRFRKKLIERWACEIADFFIKNKVGTVQMENLESMKRKEDSYFNIRLRGFWPYAEMQNKIEFKLKQYGVEIRRVAPNNTSRTCSKCGHLNNYFNFEYRRKNKFPHFKCEKCNFKEDADYNAALNISNPKLKSTKEEP

SEQ ID NO: 1281 - protein, 726 aa, synthetic construct
SEVEFSHEYWMRHALTLAKRARDEREVPVGAVLVLNNRVIGVGWNRAIGLHDPTAHAEIMALRQGGLVMRNYRLIDATLYVTFEPCIMCAGAMIHSRIGRVVFGVRNSKRGAAGSLMNVLNYPGMNHRVEITEGVLADECAALLCDFYRMPRQVLNAQKKAQSSINSGGSSGGGSGGETPGTSESATPESSGGSSGGSAKNTITKTLKLRIVRPYNSAEVEKIVADEKNNREKIALEKNKDKVKEACSKHLKVASYCTTQVERNACLFCKARKLDDKFYQRLRGQFPDAVFWQELGGIFRQLQKQAAEIYNQSLIELYYEIFIKGKGFANASSVEHYLSDVCYTRAAELFKNAAIASGLRGKVKSNFRLKELKNMKSGLPTTKSDNFPIPLVKQKGGQYTGFEISSHNGDFIIKIPFGRWQVKKEISKHRPWEKFDFEQVRKSPKPISLLLSTQRRKRNKGWSKDEGTEAEIRKVMSGDYQTSYIEVKRGSKTGEKSAWMLNLSIDVPKIDKGVDPSIIGGIDVGVKSPLVCAINNALSRYSISDKDLFHFNKKMFARRRILLKKNRHKRAGHGAKNKLKPISILTEKSERFRKKLIERWACEVADFFIKNKVGTVQMENLESMKRREDSYFNIRLRGFWPYAKMQSKIEFKLKQYGIEIRKVAPNNTSRTCSKCGHLNNYFNFEYRKKNKFPHFRCEKCNFKEDADYNAALNISNPKLKSTKEEP

SEQ ID NO: 1282 - protein, 726 aa, synthetic construct
SEVEFSHEYWMRHALTLAKRARDEREVPVGAVLVLNNRVIGEGWNRTIGLHDPTAHAEIMALRQGGLVMQNYRLTDATLYVTFEPCVMCAGAMIHSRIGRVVFGVRNSKRGAAGSLMNVLNYPGMNHCVEITEGILVDECAALLCDFYRMPRQVLNAQKKAQSSISSGGSSGGSCCSETPGASESVTPKSSGGSSAGSTKNTITKTLKLRIVRPYNSAEVEKIVADEKNNREKIALEKNKDKVKEACSKHLKVASYCTTQVERNACLFCKARKLDDKFYQRLRGQFPDAVFWQEIGEIFRQLQKQAAEIYNQSLIELYYEIFIKGRGFANASSVEHYLSDVCYTRAAELFKNAAIASGLRGKVKSNFRLKELKNMRSGLPTTKSDNFPIPLVKQKGGQYTGFEISSHNDDFIIKIPFGRWQVKKEISKHRPWEKFDFEQVRKSPKPISLLLSTQRRKRNKGWSRDEGTEAEIRKVMNGDYQTSYIEVKRGSKIGEKSAWMLNLSIDVPKIDKGVDPGIIGGIDVGVKSPLVCAINNASSRYSISDNDLFHFNKKMFARRRILLKKNRHKRAGHGAKNKLKPITIMTEKSKRFRKKLIERWACEIADFFIKNKVGTVQMENLESMKRKEDSYFNIRLRGFWPYAEMQNKIEFKLKQYGIEIRKVAPNNTSKTCSKCGHLNNYFNFEYRKKNKFPHFKCEKCNFKENADYNAALNISNPKLKSTKEEP

SEQ ID NO: 1283 - protein, 726 aa, synthetic construct
SEVEFSHEYWMRHALTLAKRARDEREVPVGAVLVLNNRVIGVGWNRAIGLHDPTAHAEIMALRQGGLVMQNYRLIDAALYVTFEPCIMCAGAMIHSRIGRVVFGVRNSKRGAAGSLMNVLNYPGMNHRVEITEGVLADECAALLCDFYRMPRQVLNAQKKAQSSINSGGSSGGGSGGETPGTSESATQESFGGSSGGSAKNTITKTLKLRIVRPYNSAEVEKIVADEKNNREKIALEKNKDKVKEACSKHLKVAAYCTTQVERNACLFCKARKLDDKFYQKLRGQFPDAVFWQEISEIFRQLQKQAAVIYNQGLIELYYEIFIKGKGIANASRVEHYLSNVCYTRAAELFKNAAIASGLRNKIKSNFRLKELRNMKSGLPTTKSDNFPIPLVRQKGGQYTGFEISNHDGDFIIKIPFGRWRVKKEINKHRPWEKFDFEQVRKSPKPISLLLSTQRRKRNKGWSKDEGTEAEIRKVMNGDYQTSYIEVKRGSKIGEKSAWMLNLSIDVPKIDKGVDPGIIGGIDVGVKSPLVCAINSASSRYSISDNDLFHFNKKMFARRRILLKKNGHKRAGHGAKNKLKPITIMTEKSKRFRKKLIERWACEIADFFIKNKVGTVQMENLESMKRREDSYFNIRLRGFWPYAEMQNKIEFKLKQYGIEIRKVAPNNTSKTCSKCGHLNNYFNFEYRKKNKFPHFKCEKCSFKENADYNAALNISNPKLKNTKEEP

SEQ ID NO: 1284 - protein, 726 aa, synthetic construct
SEVEFSHEYWMRHALTLAKRARDEREVPVGAVLVLNNRVIGEGWNRAIGLHDPTAHAEIMALRQGGLVMQNYRLTDATLYVTFEPCVMCAGAMIHSRIGRVVFGVRNSKRGAAGSLMNVLNYPGMNHCVEITEGILVDECAALLCDFYRMPRQVFNAQKKAQSSINSGGSSGGSSGSETPSTSESATPESSGGSSGGSAKNTITKTLQLRIVRPYNSAEVEKIVTDEKNNRERIALEKNKDKVKEACSKHLKMASYCTTQVERNACLFCKARKLDDKFYQKLRGQFPDAVFWQELGGIFRQLQKQAAEIYNQSLIELYYEIFIKGKGITNASRVEHYLSDVCYTRAAELFKNAAIASGLRSKVRSNFRLKELKNMKSGLPTTKSDNFPIPLVKQKGGQYTGFEISSHNSDFIIKIPFGRWQVKKEIDKYRPWEKFDFEQVRKSPKPISLLLSTQRRKRNKGWSKDEGTEAEIRKVMNGDYQTSYIEVKRGRKIGERSAWMLNLSIDVPKIDKGVDPSIIGGIDVGVKSPLVCAINNAFSRYSISDNDLFHFNKKMFARRRILLKKNRPKRAGHGARNKLKPISILTEKSGRFRKKLIERWACEIADFFIKNKVGTVQMENLESMKRKEDSYFNIRLRGFWPYAEMQNKIEFKLKQYGIEIRKVAPNNTSKTCSKCGHLNNYFNFEYRKRNKFPYFKCEKCNFKENADYNAALNISNPKLKSTKEEP

SEQ ID NO: 1285 - protein, 726 aa, synthetic construct
SEVEFSHEYWMRHALTLAKRARDEREVPVGAILVLNNRVIGVGWNRAVGLHDPTAHAEIMALRQGGLVMQNYRLIEATLYVTFEPCIMCAGAMIHSRIGRVVFGARNSKRGAAGSLMNVLNYPGMNHRVEITEGILADECAALLCDFYRMPRQVFNARKKAQSSINPGGSSGGSGGSETPGTSESPTPESSGGSSGGSAKNTITKTLKLRIVRPYNSAEVEKIVAEEKDNREKIALEKNKDKVREACSKHLKVAAYCTTQVERNACLFCKARKLDDKFYQKLRGQFPDAVFWQEIGEIFRQLQKQAAEIYNQSLIELYYEIFIKGKGFANASSVEHYLSDVCYTRAAELFKNAAIASGLRGKVKSNFRLKELKNMKSGLPTTKSDNFPIPLVKQKGGQYTGFEISNHDSDFIIKIPFGRWQAKKEIDKYRPWEKFDFEQVRKSPKPISLLLSTQRRKKNRGWSKDEGTEAEIKKVMNGDYQTSYIEVKRGSKIGEKSAWMLNLSIDVPKVDKGVDPSIIGGIDVGVKSPLVCAINNAFSRYSISDNELFHFNKKMFARRRILLKKNRHKRTGHGAKNKLKPISVLTEKSGRFRKKLIERWACEIADFFIKNKVGTVQMENLGSMKRKEDSYFNIRLRGFWPYAEMQNKIEFKLKQYGIEIRKVAPDNTSKTCSKCGHLNNYFNFEYRKKNKFPHFKCEKCNFKEDADYNAALNISNPKLKSTKEEP

SEQ ID NO: 1286 - protein, 726 aa, synthetic construct
SEVEFSHEYWMRHALTLAKRARDEREVPVGAVLVLNNRVIGEGWNRAIGLHDPTAHAEIMALRQGGLVMQNYRLTDATLYVTFEPCVMCAGAMIHSRIGRVVFGVRNSKRGAAGSLMNVLNYPGMNHRVEITEGILVDECAALLCDFYRMPCQVLNARKKAQSSISSGGSSGGSSGGDTLGASESVTPKSSVGSSASSTKNTITKTLKLRIVRPYNSAEVEKIVADEKDNREKIALEKNKDKVKEACSKHLKVAAYCTTQVERNACLFCKARKLDDKFYQKLRGQFPDAVFWQEIGEIFRQLQKQAAEIYNQSLIELYYEIFIKGKGFANASSVEHYLSDVCYTRAAELFRNAAIASGLRGKVKSNFRLKELKNMKSGLPTTKSDNFPIPLVKQKGGQYTGFEISSHNSDFIIEIPFGRWQVKEEINKYRPWEKFDFEQVRKNPKPISLLLSTQRRKRNKGWSKDEGTEAEIRKVMNGDYQTSYIEVKRGSKIGEKSAWVLNLSIDVPKIDKGVDPSIIGGIDVGVKSPLVCAINNAFSRYSISDNDLFRFNKKMFARRRILLGKNRHKRAGHGVKNKLKPITILTEKSGRFRKKLIERWACEIADFFVKNKVGTVQMENLESMKRKEDSYFNIRLRGFWPYAEMQNKIEFKLKQYGIKVRKVAPSNTSKTCSKCGHLNNYFSFEYRKKNKFPHFKCEKCNFKENADYNAALNISNPKLKSTKEEP

SEQ ID NO: 1287 - protein, 726 aa, synthetic construct
SEVEFSHEYWMRHALTLAKRARDEREVPVGAVLVLNNRVIGVGWNRAIGLHDPTAHAEIMALRQGGLVMQNYRLIDATLYVTFEPCVMCAGAMIHSRIGRVVFGVRNSKHGAAGSLVNVLNYPGMNHRVEITEGILADECAALLCDFYRMPRQVFNARKKAQSSINSGGSSGGSSGSVTPGTSESATPESSGGSSGGSAKNTITKTLKLRIVRPYNSAEVEKIVADEKNNREKIALEKNKDRVKEACSKHLKVASYCTTQVERNACLFCKARKLDDKFYQKLRGQFPDAVFWQELGEIFRQLQKQAAEIYNQSLIELYYEIFIKGKGITNASRVEHYLSDVCYARAAELFKNAAIASGLRSKVRSNFRLKELKNMKSGLPTTKSDNFPIPLVKQKGGQYTGFEISNHNSDFIIKIPFGRWQVKREIDKYRPWEKFDFEQVRKSPKPISLLLSTQRRKRNRGWSKDEGTEAEIRKVMNGDYQTSYIEVKRGSKIGEKSAWMLNLSIDVPKIDKGVDPSIIGGIDVGVKSPLVCAINNALSRYSISDNDLFHFNKRMFARRRILLRGNRHKRAGHGAKNKLKPITILTEKSKRFRKKLIERWACEIADFFIKNKVGTVQMENLESMKRKEDSYFNIRLRGFWPYAEMQNKIELKLKQYGIKIRKVAPNNTSKTCSKCGHLNDYFNFEYRKKNKFPHFKCEKCNFKEDADYNAALNISNPKLKSTREEP

SEQ ID NO: 1288 - protein, 726 aa, synthetic construct
SGVEFSHEYWMRHALTLAKRARDEREVPVGAILVLNNRVIGEGWNRAIGLHDPTAHAEIMALRQGGLVMQNYRLIDATLYVTFEPCVMCAGAMIHSRIGRVVFGVRNNKHGAAGSLVNVLDYPGMNHRVEITEGILADECAALLCDFYRMPRQVLNAQKKAQSSISSGGSSGSSSGSETPGASESVTPKGSGGSSAGSTKNTITKTLKLRIVRPYNSAEVEKIVADEKNNREKIALERNRDKVKEACSKHLEVAAYCTTQVERNACLFCKARKLDDKFYQKLRGQFPDAVFWQELGEIFRQLQKQAAEIYNQSLIELYYEIFIKGKGITNASRVEHYLSDVCYTRAAELFKNAAIASGLRSKVRSNFRLKELKNMKSGLPTTKSDNFPIPLVKQKGGQYTGFEISNRNSDFVIKIPFGRWQVKKEINKYRPWEKFDFEQVRKSPKPISLLLSTQRRKRNKGWSKDEGTEAEIRKVMNGDYQTSYIEVKRGSRIGEKSAWMLSLSIDVPKIDRGVDPSIIGGIDVGVKSPLVCAINNAFSRYCISDNDLFHFNKKMFARRRILLKKNGRKRAGHGAKNKLKPISILTGKSERFRKKLIERWACEIADFFIKNKVGTVQMENLESMKRKEDSYFNIRLRGFWPYAEMQNKIEFKLKQYGIEIRKVAPNNTSKTCSKCGHLNNYFNFEYRKKNKFPHFKCEKCNYKENADYNAALNISNPKLKSTKEEP

SEQ ID NO: 1289 - protein, 726 aa, synthetic construct
SEVEFSHEYWMRHALTLAKRARDEREVPVGAILVLNNRVIGEGWNRAIGLHDPTAHAEIMALRQGGLVTQNYRLIDATLYVTFEPCAMCAGAMVHSRIGRVVFGVRNSKRGAAGSLMNVLNYPGMDHRVEITGGILADECAALLCDFYRMPRRVFNAQKKAHSSINSGGSSGGSSGSVTPGTSESATPESSGGSSGGPAKNTITKTLKLRIVRPYNSAEVEKIVADEKNNREKTALEKNKDKVKEACSKHLKVAAYCTTQVERNACLFCKARKLDDKFYQKLRGQFPDAVFWQEVGEIFRQLQKQAAEIYNQSLIELYYEIFIRGKGFANASSVEHYLSDVCYTRAAELFKNAAIASGLRGKVKSNFRLKELKNMKSGLPTTKSDNFPIPLVKQKGGQYTGFEISNHNSDFIIKIPFGRWQVKKEINKYRPWEKFDFEQVRKSPKPISLLLSTQRRKRNKGWNKDEGTEAEIRKVMNGDYQTSYIEVKRGSRIGEKSAWMLSLSIDVPKIDRGVDPSIIGGIDVGVKSPLVCAINNALSRYSISDNDLFHFNKKMFARRRILLKKNRHRRAGHGAKNKLKPITIMTEKSKRFRKKLIERWACEIADFFIKNKVGTVQMENLESMKRKEDSYFNIRLRGFWPYAEMQNKIEFKLRQYGIEVRKVAPNNTSKTCSRCGHLNNYFNFEYRKKNKFPHFKCEKCNFKENADYNAALNISNPKLKGTKEEP

SEQ ID NO: 1290 - protein, 726 aa, synthetic construct
SEVEFSHEYWMRRALTLAKRARDEREVPVGAVLVLNNRVIGVGWNRAVGLHDPTAHAEIMALRQGGLVMQNYRLTEATLYVTFEPCTMCAGAMIHSRIGRVVFGVRNSKRGAAGSLMNVLNYPGMNHRVEITEGILADECAALICDYYRMPRQVFNARKKAQSSINSGGSSDGGSGSETPGTSESATPESSGGSSGGSAKNTITKTLKLRIVRPYNSAEVEKIVADEKNNREKIALEKNKDKVKEACSEHLKVAAYCTTQVERSACLFCKARKLDDKFYQKLRGQFPDAVFWQEIGEIFRQLQKQAAEIYNQSLIELYYEIFIKGKGFANASSVEHYLSDVCYTRAAELFKNAAIASGLRGKVKSNFRLKELKNMRSGLPTTKSDNFPIPLVKQKGGQYTGFEISNHDGDFIIKIPFGRWQVKREIDKYRPWEKFDFEQVRKSPKPISLLLSTRRRKRNKGWSKDEGTEAEIRKVMNGDYQTSYIEVKRGSKIGEKSAWMLNLSIDVPKIDKGVDPSIIGGVDVGVKSPLVCAINNAFSRYSISDNDLFRFNKRMFARRRILLKRNRHKRAGHGAKNKLKPISILTEKSGRFRKKLIERWACEIANFFIKNKVGTVQMENLESMKRKEDSYFNIRLRGFWPYAEMQNKIEFKLKQYGIKIRKVAPNNTSKTCSKCGHLNNYFSFEYRKKNKFPHFKCEKCNFKEDADYNAALNISNPKLKSTKEEP

SEQ ID NO: 1291 - protein, 726 aa, synthetic construct
SEVEFSHEYWMRHALSLAKRARDEREVPVGAVLVLNNRIIGEGWNRVIGLHDPTAHAEIMALRQGGLVMQNYRLTDATLYVTFEPCVMCAGAMVHSRIGRVVFGVRNSKRGAAGSLMNVLNYPGVNHCVEITEGILVDECAALLCDFYRMPRQVLNAQKKAQSSINSGGSSGGSSGSETPGTSESPTPESSVGSSAGSTKNTITKTLKLRIVRPYNSAEVEKIVADEKNNREKIALEKNKDKVKEACSKHLKVAAYCTTQVERNACLFCKARKLDDKFYQKLRGQFPDAVFWQELGEILRQLQKQAAEIYNQSLIELYYEIFIKGKGFANASSVEHYLSDVCYTRAAELFKNAAIASGLRGKVKSNFRLKELKNMKSGLPTTKSDNFPIPLVKQKGGQYTGFEISSHNDDFIIKIPFGRWQVKKEIDKYRPWEKFDFEQVRKSPKPISLLLSTQRRKRNKGWSKDEGTEAEIRKVMNGDYQTSYIEVKRGGKIGEKSAWMLNLSIDVPKIDKGVDPSIIGGIDVGVRSPLVCAINNAFSRYSISDNDLFRFNKKMFARRRILLKKNRHKRAGHGAKNKLKPITILTGKSRRFRKKLIERWACEIADFFIKNKVGTVQMESLESMKRKEDSYFNIRLRGFWPYAEMQNKIEFKLKQYGIKIRKVAPNNTSKTCSKCGHLNNYFSFEYRKKNKFPHFKCEKCNFKESADYNAALNISNPKLKSTKEEP

SEQ ID NO: 1292 - protein, 726 aa, synthetic construct
SEVEFSHEYWMRHALTLAKRARDEREVPVGAVLVLNNRVIGVGWNRAIGLHDPTAHAEIMALRQGGLVMQNYRLIDATLYVTFEPCVMCAGAMIHSRIGRVVFGVRNSKHGAAGSLVNVLNYPGMNHRVEITEGILADECAALLCDFYRMPRQVFNARKKAQSSINSGGSSGGSSGSETPGTSESATPKSSGGSSGGSAKNTITKALKLRIVRPYNSAEVEKIVADEKNNRERIALEKNKDKVKEACGKHLKVAAYCTTQVERNACLFCKARKLDDKFYQKLRGQFPDAVFWQEIGEIFRQLQKQAAEIYNQSLIELYYEILIKGKGFANASSVEHYLSDVCYTRAAELFKNAAIASGLRGKVKSNFRLKELKNMRSGLPTTKSDNFPIPLVKQKGGQYAGFEISSHNDDFIIKIPFGRWQVKKEIDKYRPWEKFDFEQVRKSPKPISLLLSTRRRKRNKGWSKDEGTEAEIRKVMNGDYQTSYIEVKRGSKTGEKSAWMLNLSIDVPKIDKGVDPSIIGGIDVGVKSPLVCAINNALSRYSISDNDLFHFNKKMFARRRILLKKNRRKRAGHGAKNKLKPISILTEKSERFRKKLIERWACEIADFFIKNKVGTVQMENLESMKRREDSYFNIRLRGFWPYAKMLNKIEFKLKQYGIKIRKVAPNNTSKTCSKCGHLNNYFNFEYRKKNKFPHFKCEKCNFKENADYNAALNISNPKLKSTKEEP

SEQ ID NO: 1293 - protein, 726 aa, synthetic construct
SEVEFSHEYWMRHALSLAKRARDEREVPVGAVLVLNNRVIGEGWNRAIGLHDPTAHAEIMALRQGGLVMQNYRLTDATLYVTFEPCVMCAGAMIHSRIGRVVFGVRNSKRGAAGSLMNVLNYPGMNHCVEITEGILVDECAALLCDFYRMPRQVLNAQKKAQSSISSGGSFGGSGGGETPGASESVTPKSSGGSSAGSTKNTITKTLKLRIVRPYNSAEVEKIVADEKNSREKIALEKNKDKVKEACSEHLKVAAYCTTQVERSACLFCRARKLDDGFYQKLRGQFPDAVFWQETGEIFRQLQRQAAEIYNQSLIELYYEIFIKGKGFANASSVEHYLSDVCYTRAAELFKNAAIASGLRGKVKSNFRLKELKNMKSGLPTTKSDNFPIPLVKQKGGQYTGFEISSHNDDFIIKIPFGRWQVKKEIDRYRPWEKFDFEQVRKSPKPISLLLSTQRRKRNKGWSKDEGTEAEIRKVMNGDYQTSYIEVKRGSKIGEKSAWMLNLSIDVPKIDKGVDPSIIGGIDVGVKSPLVCAINNTIGRYSISDNDLFRFNKKMFARRRILLKKNRHKRAGHGAKNKLKPISILTEKSGRFRKKLIERWACEIADFFIKNKVGTVQMENLESMKRKEDSYFNIRLRGLWPYAEMQNKIEFKLKQYGIEIRKVAPNNTSKTCSKCGHLNNYFSFEYRKKNKFPHFKCEKCNFKENADYNAALNISNPKLKSTKEEP

SEQ ID NO: 1294 - protein, 726 aa, synthetic construct
SGVEFGHEYWMRHALTLARRARDEGEVPVGAVLVLNNRVIGEGWNRAIGLHDPTAHAEIMALRQGGLVMQNYRLVDATLYVTFEPCVLCAGAMVHSRIGRVVFGVRNSKRGAAGSLMNVLNHPGMNHRVEITGGILADECAALLCDFYRMPRQVFNAQKKARSNINSGGSSGGSSGSETLGTSESATPESSGGSSGGSAKNTITKTLKLRIVRPYNSAEVEKIVADEKNNREKIALEKNKDKVKEACSEHLKVAAYCTTQVERNACLFCKARRLDDKFYQKLRGQFPDAVFWQELGEILRQLQKQAAEIYNQSLIELYYEIFIKGRGFANASSVEHYLSDVCYTRAAELFKNAAIASGLRGKVKSNFRLKELKNMKSGLPTTKSDNFPIPLVKQKGGQYTGFEISSHNDDFIIKIPFGRWQVKKEIDKYRPWEKFDFEQVRKSPKPISLLLSTQRRKRNKGWSKDEGTEAEIRKVMNGDYQTSYIEVKRGSKTGEKSAWMLNLSIDVPKIDKGVDPSIIGGIDVGVKSPLVCAINNAFSRYSISDNDLFHFNKKMFARRRILLKKNRRRRAGHGVKNKLKPITILTEKSGRFRKKLIERWACEIADFFVKNKVGTVQMENLESMKRKEDSYFNIRLRGFWPYAEMQNKIEFKLKQYGIKVRKVAPNNTSKTCSKCGHLNNYFSFEYRKKNKFPHFKCEKCNFKEDADYNAALNISNPKLKSTKEEP

SEQ ID NO: 1295 - protein, 726 aa, synthetic construct
SEVEFSHEYWMRHALTLAKRARDEREVPVGAILVLNNRVIGEGWNRAIGLHDPTAHAEIMALRQGGLVMQNYRLIDATLYVTFEPCVMCAGAMIHSRIGRVVFGVRNSKRGAAGSLMNVLNYPGMGHRVEITEGILAGECAALLCDFYRMPRQVFNAQKKAQSNINSGGSSGGNSGSEAPGTSESPTPESPGGSSGGSAKNTITKTLKLRIVRPYNSAEVEKIVADEKNNREKIALEKNKDKVKEACSKHLKVVAYCTTQVERNACLFCKARKLDDKFYQKLRGQFPDAVFWQEIGEIFRQLQKQAAEIYNQSLIELYYEIFIKGRGFANASSVEHYLSDVCYTRAAELFKNAAIASGLRGKVKSNFRLKELKNMKSGLPTTKSDNFPIPLVKQKGGQYTGFEISSHNDDFIIKIPFGRWQAKKEIDKYRPWEKFDFEQVRKSPKPISLLLSTQRRKRNKGWSKDEGTEAEIRKVMNGDYQTSYIEVKRGSKIGEKSAWMLNLSIDVPKIDKGVDPSIIGGIDVGVKSPLVCAINNACSRYSISDNDLFHFNKKMFARRRILLKKNRHKRAGHGAKNKLKPITILTEKSKRFRKKLIERWACEIADFFIKNKVGTVQMENLESMKRKEDSYFNTRLRGFWPYAEMQNKIEFKLKQYGIEIRKVAPNNTSKTCSKCGHLNNYFSFEYRKKNKFPHFKCEKCNFKENADYNAALNISNPKLKSTKKEP

SEQ ID NO: 1296 - protein, 726 aa, synthetic construct
SEVEFSHEYWMRHALTLAKRARDGREVPVGAVLVLNNRVIGEGWNRAIGLHDPTAHAEIMALRRGGLVMQNYRLIDATLYVTFEPCVMCAGAMVHSRIGRVVFGVRNSKRGAAGSLMNVLDYPGMGHRVEITEGILADECAALLCDFYCMPRQVFNAQKRAQSSINSGGLSGGSSGSDTPGTSESATPESSGGSSGGSAKNTITKTLKLRIVRPYNSAEVEKIVADEKNNREKIALEKNKDKVKEACSKHLKVAAYCTTQVERNACLFCKARKLDDKFYQKLRGQFPDAVFWQEISEIFRQLQKQAAEIYNQSLIELYYEILIKGKGIANASRVEHYLSDVCYTRAAELFKNAAIASGLRSKIKSNFRLKELRNMKSGLPTTKSDNFPIPLVKQKGGQCTGFEISNHNSDFIIKIPFGRWQVKKEIDKYRPWEKFDFEQVRKSPKPISLLLSTQRRKRNKGWSKDEGTEAEIRKVMNGDYQTSYIEVKRGSKTGEKSAWMLNLSIDVPKIDKGVDPSIIGGIDVGVRSPLVCAINNAFSRYSISDNDLFRFNKKMFARRRILLKKNRHKRAGHGAKNKLKPISILTGKSERFRKKLIERWACEIADFFIKNKVGTVQMENLESMKRKEDSYFNIRLRGFWPYAEMQNKIEFKLKQYGIEIRKVAPNDTSKTCSKCGHLNNYFNFEYRKKNKFPHFKCEKCNFKENADYNAALNISNPKLKSTKGEP

SEQ ID NO: 1297 - protein, 726 aa, synthetic construct
SEVEFSHEYWMRHALTLAKRARDEREVPVGAVLVLNNRAIGEGWNRAIGLHDPTAHAEIMALRQGGLVMQNYRLTDATLYVTFEPCVMCAGAMIHSRIGRVVFGVRNSKRGAAGSLMNVLNYPGMNHCVEITEGILVDECAALLCDFYRMPRQVLNAQKKAQSSISSGGSSGGSSSSETPGTSGSATPESPGGSSGGSAKSTITKTLKLRIVRPYNSAEVEKIVADEKNNREKIALEKNKDKVKEACSKHLKVAAYCTTQVERNACLFCKARRLDDKFYQKLRDQFPDAVFWQEIGEIFRQLQKQAAEIYNQSLIELYYEIFIKGKGLANASSVEHYLSDVCYTRAAELFKNAAIASGLRGKVKSNFRLKELKNMKSGLPTTKSDNFPIPLVKQKGGQYTGFEINSHNDDFIIKIPFGRWQVKKEIDKYRPWEKFDFEQVRKSPKPISLLLSTQRRKRNKGWSKDEGTEAEIRKVMNGDYQTSYIEVKRGSKTGEKSAWMLNLSIDVPKIDKGVDPSIIGGIDVGVKSPLVCAINNAFSRYSISDNDLFRFNKKMFARRRILLGKNRHRRAGHGAKNKLKPISILTEKSKRFRKKLIERWACEIADFFIKNKVGTVQMENLESMKRREDSYFNIRLRGFWPYAEMQNKIEFKLKQYGIEIRKVAPNNTSKTCSKCGHLNNYFNFEYRKKNKFPHFKCEKCNFKENADYNAALNISNPKLKSTKEEP

SEQ ID NO: 1298 - protein, 726 aa, synthetic construct
SEVEFSHEYWMRRALTLAKRARDEREVPVGAVLVLNNRVIGVGWNRAVGLHDPTAHAEIMALRQGGLVMQNYRLIDATLYVTFEPCVMCAGAMVHSRIGRVVFGVRNSKRGAAGSLMNVLDYPGMDHRVEITGGILADECAALLCDFYRMPRQVFNAQKKAQSSINSGGSSGGSSGSETPGASGSVIPRSSGGSSAGSTKDTITKTLKLRIVRPYNSAEVEKVVADEKNNREKIAMEKNKDKVKEACSKHLKVASYCTTQVERNACLFCKARKLDDKFYQKLRGQFPDAVFWQELGGIFRQLQKQAAEIYNQSLIELYYEIFIKGKGITNASRVEHYLSDVCYTRAAELFKNAAIASGLRSKVRSNFRLKELKNMKSGLPTTKSDNFPIPLVKQKGGQYTGFEISSHNSDFIIKIPFGRWQEKEEIDKYRPWEKFDFEQVRRSPKPISLLLSTQRRKKNKGWSKDEGTEAEIRRVMNGDYQTSYIEVKRGSKIGEKSAWMLNLSIDVPKIDKGVDPSIIGGIDVGVKSPLVCAINNAFSRYSISDNDLFRFNKKMFARRRILLKKNRHQRAGHGAKNKLKPITILTEKSGRFRKKLIERWACEIADFFIKNKVGTVQMENLESMKRKEDSYFNIRLRGFWPYAEMQNKIEFKLKQYGIKIRKVAPNNTSKTCSKCGHLNNYFSFEYRKKNKFPRFKCEKCNFKENADYNAALNISNPKLMSTKEEP

SEQ ID NO: 1299 - protein, 726 aa, synthetic construct
SEVESSHEYWMRHALTLAKRARDEREVPVGAVLVLNNRVIGEGWNRAIGLHDPTAHAEIMALRQGGLVMQNYRLIDATLYVTFEPCVMCAGAMIHSRIGRVVFGVRNNKHGAAGSLVNVLNYPGMNHRVEITEGILADECAALLCDFYRMPRQVFNARKKAQSSINPGGSSGGSSGSETPGTSESATPESSGGGSSGSAKNTITKTLQLRIVRPYNSAEVEKVVADEKNNREKIALEKNKDKVKEACSKHLKVASYCTTQVERNACPFCKARKLDDKFYQKLRGQFPDAVFWQELGEILRQLQKQAAEIYNQSLIELYYEIFIKGKGFANASSVEHYLSDVCYTRAAELFKNAAIASGLRGKVKSNFRLKELKNMKSGLPTTKSDNFPIPLVKQKGGQYTGFEISSHNDDFIIKIPFGRWQVKEEIDKYRPWEKFDFEQVRKNPKPISLLLSTQRRKRNKGWSKDEGTEAEIRKVMNGDYQTSYIEVKRGSKIGEKSAWMLSLSIDVPKIDKGVDPSIIGGIDVGVKSPLVCAINDAFSRYSISDNDLFHFNKKMFARRRILLKKNRHKRAGHGAKNKRKPISILTEKNERFRKKLIERWACEIADFFIKNKVGTVQMENLESMKRKEDSYFNIRLRGFWPYAEMQNKIEFKLKQYGIEIRKVAPNNTSKTCSKCGHLNNYFNFEYRKKNKFPHFKCEKCNFKENADYNAALNISNPKLKSTKEEL

SEQ ID NO: 1300 - protein, 726 aa, synthetic construct
SEVEFSHEYWMRHALTLAKRARDEREVPVGAVLVLNNRVIGEGWNRAIGLHDPTAHAEIMALRQGGLVMQNYRLIDATLYVTFEPCVMCAGAMVHSRIGRVVFGVRNSKRGAAGSLMNVLDYPGMGHRVEITEGILADECAALLCDFYRMPRQVFNAQKRAQSSINSGGSSGGSSGSETLGASESATPESSGGGSSGSAKNTITKTLQLRIVRPYNSAEVEKIVADEKNNREKIALEKNKDKVREACSKHLKVAPYCTTQVERNACPFCKARKLDDKFYQKLRGQFPDAVFWQELGEILRQLQKQAAEIYNQSLIELYYEIFIKGRGFANASSVEHYLSDVCYTRAAELFKNAAIASGLRGKVKSNFRLKELKNMKSGLPTTKSDNFPIPLVKQKGGQYTGFEISSHNDDFIIKIPFGRWQVKKEIDKYRPWEKFDFEQVRKSPKPISLLLSTQRRKRNKGWSKDEGTEAEIRKVMNGDYQTSYIEVKRGSKIGEKSAWMLNLSIDVPKIDKGVDPSIIGGIDVGVKSPLVCAINNAFSRHSISDNDLFRFNKKMFARRRILLKKNRHKRAGHGAKNKLKPISILTEKSERFRKKLIERWACEIADFFIKNKVGTVQMENLESMKRKEDSYFNIRLRGFWPYAEMQNKIEFKLKQYGIEIRKVTPNNTSKTCSRCGHLNNYFNFEYRKKNKFPHFKCEKCNFKENADYNAALNISNPKLKSSKEEP

SEQ ID NO: 1301 - protein, 726 aa, synthetic construct
SEDEFSHEYWMRHALTLAKRARDGREVPVGAVLVLNNRVIGEGWNRAIGLHDPTAHAEIMALRQGGLVMQNYRLTGATLYVTFEPCVMCAGAMIHSRIGRVVFGARNSKRGAAGSLMNVLNYPGMNHCVEITEGILVDECAALLCDFYRMPRQVLNAQKKAQSSISSGGSSGGSSGSETPGAGESTTPKSSGGSSAGSTKNTITKTLQLRIVRPYNSAEVEKIVADEKNNREKVALEKNKDKVREACSEHLKVAAYCTTQVERNACLFCKARRLDDKFYQKLRGQFPDAVFWQEIGEVFRQLQKQAAEIYNQSLIELYYEIFIKGKGFANASSVEHYLSDVCYTRAAELFKNAAIASGLRGKVKSNFRLKELKNMKSGLPTTKSDNFPIPLVKQKGGQYTGFEISSHNDDFIIKIPFGRWQVKKEIDKYRPWEKFDFEQVRKSPKPISLLLSTQRRKRNKGWGKDEGTEAEIKRVMNGDYQISYIEVKRGSKIGKKSAWMLSLSVDVPKIDKGVDPSIIGGIDVGVKSPLVCAINNALSRYSISDNDLFHFNKKMFARRRILLRNNRHKRAGHGAKSKLKPITILTEKGERFRKKLIERWACEIANFFIKNKVGTVQMENLESMKRKEDSYFNVRLRGFWPYAEMQNKIEFKLKQYGIEIRKVAPNNTSKTCSRCGHLNNYFNFEYRRKNKFPHFKCEKCNFKENADYNAALNISDPKLKSTKEEP

SEQ ID NO: 1302 - protein, 726 aa, synthetic construct
SEVEFSHEYWMRHALTLAKRARDEREVPVGAVLVLNNRVIGEGWNRAIGLHDPTAHAEIMALRQGGLVMQNYRLTDATLYVTFEPCVMCAGAMIHSRIGRVVFGVRNGKRGAAGSLMNVLNYPGMNHRVEITEGILADECAALLCDFYRMPRQVFNAQKKAQSSIDSGGLSGGSSGSETPGTSESTTPGSSGGSSGGSAKDTITKTLKLRIVRPYNSAEVEKIVADEKNNREKIALEKNKDKVKEACSKHLKVATYCTTQVERNACLFCKARRLDDKFYQKLRGQFPDAVFWQEISEIFRQLQKQAAEIYNQSLIELYYEVFIKGKGIANAGSVEHYLSDVCYTRAAELFKNAAIASGLRNKIKSNFRLKELRNMKSGLPTTKSDNFPIPLVRQKGGQYTGFEISNHNSDFIIKIPFGRWQVKEEIDRYRPWEKFDFAQVRKSPKPISLLLSTQRRKRNRGWSKDESTEAEIKKVMNGDYQTSYIEVRRGSKIGEKSAWMLNLSIDVPKIDKGVDPSIIGGIDVGVKSPLVCAISNAFSRYSISDNDLFRFNKKMFARRRILLKKNRHKRAGHGAKNKLKPISILTGKSERFRKKLIERWACEIADFFIKNKVGTVQMENLESMKRKEDSYFNIRLRGFWPYAEMQNKIEFKLKQYGIEIRKVAPNNTSKTCSKCGHLNNYFNFEYRKKNKFPHFKCEKCNFKENADYNAALNISNPKLKSTKEKP

SEQ ID NO: 1303 - protein, 726 aa, synthetic construct
SEVEFSHEYWMRHALTLAKRARDEREVPVGAVLVLNNRVIGEGWNRAIGLHDPTAHAEIMALRQGGLVMQNYRLINATLYVTFEPCVMCAGAMIHSRIGRVVFGVRNSKHGAAGSLMNVLNYPGMNHRVEITEGILADECAALLCDFYRMPRQVFSARKKAQSSINSGGSSGGNSGNKTPGTSESATPESSGGSSGGSAKNTITKTLKLRIVRPYNSAEVEKIVADEKNNREKIALEKNKDKVEEACSKHLKVASYCTTQVERNACLFCKARKLDDKFYQKLRGQFPDAVFWQELGEILRQLQKQAAEIYNQSLIELYYEIFIKGRGFANASSVEHYLSDVCYTRAAELFKNAAIASGLRGKVKSNFRLKELRNMRGGLPTTKSDNFPIPLVKQKGGQYTGFEISSHNDDFIIKIPFGRWQVKKEIDKYRPWEKFDFEQVRKSPKPISLLLSTQRRKRNKGWSKDEGTEAEIRKVMNGDYQTSYIEVKRGSKIGEKSAWMLNLSIDVPKIDKGVDPSIVGGIDVGVKSPLVCAIDNTLSRYSISDNDLFHFNKKMFARRRILLKKNRHRRAGHGAKNKLKPISILTEKSKRFRKKLIERWACEIADFFIKNKVGTVQMENLESMKRKEDSYFNIRLRGFWPYAEMQNKIEFKLKQYGIEIRKVAPNNTSKTCSKCGHLNNYFDFEYRKKNKFPHFKCEKCNFKENADYNAALNISNPMLKSTKGEP

SEQ ID NO: 1304 - protein, 726 aa, synthetic construct
SEVEFSHEYWMRHALTLAKRARDEREVPVGAVLVLNNRVIGEGWNRAIGLHDPTAHAEIMALRQGGLVMQNYRLADATLYVTFEPCVLCAGAMVHSRIGRVVFGVRNSKRGAAGSLMNVLNYPGMNHRVEITEGILADECAALLCDFYRMPRHVLNAQKKAQSSISSGGSSGGCSGSETPGASESVTPKSSGGSSAGSTKNTITKTLKLRIVRPYNSAEVEKIVADEKNSREKIALERNKDKVKEACSEHLKVAAYCTTQVERNACLFCKARKLDDRFYQKLRGQFPDAVFWQETGEIFRQLQRQAAEIYNQSLIELYYEIFIKGKGFANASSVEHYLSDVCYTRAAELFKNAAIASGLRGKVKSNFRLKELKNMKSGLPTTKSDNFPIPLVKQKGGQYTGFEISSHNDDFIIKIPFGRWQVKKEIDRYRPWEKFDFEQVRKSPKPISLLLSTQRRKRNKGWSKDEGTEAEIRKVMNGDYQTSYIEVKRGSKTGEKSAWMLNLSIDVPKIDKGVDPSIIGGIDVGVKSPLVCAISNAFSRYSISDNDLFHFNKKMFARRRILLKKSKHKRAGHGAKNKLKPITILTEKSRRFRKKLIERWACEIADFFIKNKVGTVQMENLESMKRREDSYFNIRLRGFWPYAEMQNKIEFKLKQYGIEIRKVAPNNTSKTCSKCGHLNNYFNFEYRKKNKFPHFKCEKCNFKENADYNAALNISNPKLKSTKEEP

SEQ ID NO: 1305 - protein, 726 aa, synthetic construct
SEVEFSHEYWMRHALTLAKRARDEREVPVGAILVLNNRVIGEGWNRAIGLHDPTAHAEIMALRQGGLVMQNYRLIDATLYVTFEPCVMCAGAMIHSRVGRVVFGVRNSKHGAAGSLMNVLNYPGMNHRVEITEGILADECAALLCDFYRMPRQVFNARKKAQSSINPGGSSGGNSGSETPGTSESATPESSGGSSGSSAKNTITKTLKLRIVRPYNSAEVEKIVADEKNNREKIALEKNKDKVKEACSKHLKVAAYCTTQVERNACLFCKARKLDDKFYQKLRGQFPDAVFWQELGEIFRQLQKQAAEIYNQSLIELYYEIFIKGKGFANASSVEHYLSDVCYTRAAELFKNAAIASGLRGKVKSNFRLKELKNMKSGLPTTKSDNFPIPLVKQKGGQYTGFEISSHNDDFIIKIPFGRWQVKEEIDKYRPWEKFDFEQVRKSPKPISLLLSTQRRKRNKGWSKDEGTEAEIRKVMNGDYQTSYIEVKRGSKIGEKSAWMLNLSIDVPKIDKGVDPSIIGGIDVGVKSPLVCAINNAFIRYSISDNDLFHFNKKMFARRRILLKKNRHKRAGHGAKNKLKPISILTEKSKRFRKKLIERWACEIADFFIKNKVGTVQMENLESMKRKEDSYFNIRLRGFWPYAEMQNKIEFKLKQYGIEIRKVAPNNTSKTCAKCGHLNNYFNFEFRKKNKFPHFKCEKCNFKENADYNAALNISNPQLKSTKGEP

SEQ ID NO: 1306 - protein, 726 aa, synthetic construct
SEVEFSHEYWMRRALTLAKRARDEREVPVGAVLVLNNRVIGVGWNRAVGLHDPTAHAEIMALRQGGLVMQNYRLIEATLYVTFEPCIMCAGAMIHSRIGRVVFGVRNSKRGAAGSLMNVLNYPGMNHRVEITEGILADECAALLCDFYRMPRQVFNARKKAQSSINSGGSSGGSSGSETPGTSESATPKSSGGSSGGSAKNTITKALKLRIVRPYNSAEVEKIVADEKNNREKVALEKNKDKVKEACSKHLKVASYCTTQVERNACLFCKARKLDDKFYQKLRGQFPDAVFWQELGEIFRQLQKQAAEIYNQSLIELYYEIFIKGKGFANASSVEHYLSDVCYTRAAELFKNAAIASGLRGKVKSNFRLKELKNMKSGLPTTKSDNFPIPLVKQKGGQYTGFEISSHNDDFIIKIPFGRWQVKKEIDKYRPWEKFDFEQVRKSPKPISLLLSTQRRKRNKGWSKDEGTEAEIRKVMNGDYQTSYIEVKRGSKIGEKSAWMLNLSIDVPKIDKGVDPSIIGGIDVGVKSPLVCAINNAFSRHSISDNDLFRFNKKMFARRRILLGKNRHKRAGHGVKNKLKPITILTEKGGRFRKKLIERWACEIADFFVRNKVGTVQMENLESLKRKEDSYFNIRLRGFWPYAEMQNKIEFRLKQYGIKVRKVAPNNTSKTCSKCGHLNSYFNFEYRKKNKFPHFKCEKCNFKENADYNAALNISNPKLKSTKEEP

SEQ ID NO: 1307 - protein, 726 aa, synthetic construct
SEVEFSHEYWMRHALSLAKRARDEREVPVGAVLVLNNRIIGEGWNRAIGLHDPTAHAEIMALRQGGLVMQNYRLTDATLYVTFEPCVMCAGAMVHSRIGRVVFGVRNSKRGAAGSLMNVLNYPGVNHCVEITEGILVDECAALLCDFYRMPRQVLNAQKKAQSSISPGGPSGGSSGSETPGTSESAAPESSGGSSGGSAKNTITKTLKLRIVRPYNSAEVEKIVADEKNNREKIALEKNKDKVKEACSKHLRVAAYCTTRVERNACLFCKARRLDDKFYQKLRGQFPDAVFWQELGGIFRQLQKQAAEIYNQSLVELYYEILIKGKGITNASRVEHYLSDVCYTKAAELFKNAAIASGLRGKVKSNFRLKELKNMKSGLPTTKSDNFPIPLVKQKGGQYTGFEISSHNDDFIIKIPFGRWQAKKEIDKYRPWEKYDFEQVRKSPKPISLLLSTQRRKRNKGWSRDEGTEAEIRKVMNGDYQTSYIEVKRGRKIGEKSAWMLNLSIDVPKIDKGVDPSIVGGIDVGVKSPLVCAINSALGRYSISDNDLFHFNKKMFARRRILLKKNGHKRAGHGARNKLKPITVLTEKSKRFRKKLIERWACEIANFFIKNRVGTVQMENLESMKRKEDSYFNIRLRGFWPYAEMQNRIEFKLKQYGIEIRKVAPNNTSKTCSKCGHLNNYFNFEYRKKNKFPHFKCEKCNFKENADYNAALNICNPKLKGTKEEP

SEQ ID NO: 1308 - protein, 726 aa, synthetic construct
SEVEFSHEYWMRHALSLAKRARDEREVPVGAVLVLNNRVIGEGWNRAIGLHDPTAHAEIMALRQGGLVMQNYRLTDATLYVTFEPCVMCAGAMVHSRIGRVVFGVRNSKRGAAGSLMNVLNFPGMSHCVEITEGILVDECAALLCDFYRMPRQVLNAQKKAQSSISSGGSSGGSGGGETPGASESVTPKNSGGSSASSTKNTITKTLKLRIVRPYNSAEVEKIVADEKNSREKIALEKNKDKVKEACSEHLKVAAYCTTQVERNACLFCKARKLDDKFYQKLRGQFPDAVFWQELGGILRQLQKQAAEIYNQSLIELYYEIFIKGRGFANANSVEHYLSDVCYTRAAELFKNAAIASGLRGKVKSNFRLKELKNMKSGLPTTKSDNFPIPLVKQKGGQYTGFEISSHNSDFIIKIPFGRWQEKEEIDKYRPWEKFDFEQVRRSPKPISLLLSTQRRKKNKGWSKDEGTEAEIRRVMNGDYQTSYIEVKRGSKIGERSAWMLNLSIDVPKIDKGVDPSIIGGIDVGVKSPLVCAINNAFSRYSISDNDLFHFNKKMFARRRILLKKNRRRRAGHGAKNKLKPITILTEKSVRFRKKLIERWACEIADFFIKNKVGTVQMENLESMKRKEDSYFNIRLRGFWPYAEMQNKIEFKLKQYGIEIRRVAPNNTSRTCSKCGHLNNYFNFEYRRKYKFPHFKCEKCNFKEDADYNAALNISNPKLKSTKEEP

SEQ ID NO: 1309 - protein, 726 aa, synthetic construct
SEVEFSHEYWMRHALTLAKRARDEREVPVGAVLVLNNRVIGVGWNRAVGLHDPTAHAEIMALRQGGLVMQNYRLIEATLYVTFEPCIMCAGAMIHSRIGRVVFGVRNSKRGAAGSLMNVLNYPGMNHRVEITEGILADECAALLCDYYRMPRQVFNARKKVQSSINSGGSSDGGSSSETPGTSESATPESSGGSSGGSAKNTITKTLKLRIVRPYNSAEVEKIVADEKDNREKIALEKNRDKVKEACSEHLKVAAYCTTQVERSACLFCKARKLDDKFYQKLRSQFPDAVFWQEIGEIFRQLQKQAAEIYNQSLIELYYEIFIKGKGIANASSVEHYLSDVCYTRAAELFKNAAIASGLRNKIKSNFRLKELRNMKSGLPTTKSDNFPIPLVRQKGGQYTGFEISNHNGDFIIKIPFGRWQVKKEISKHRPWEKFDFEQVRKSPKPISLLLSTQRRKRNKGWSKDEGTEAEIEKVMNGDYQTSYIEVKRGSKTGGKSAWMLNLSIDVPKIDKGVDPSIIGGIDVGVKSPLVCAINNALSRYSISDNDLFHFNKKMFARRRILLRKNRHKRAGHGAKNKLKPITIMTEKSKRFRKKLIERWACEIADFFIKNKVGTVQMENLESMKKKEDSYFNIRLRGFWPYAEMQNKIEFKLKQYGIVVRKVAPNNTSKTCSKCGHLNNYFNFEYRKKNKFPHFKCEKCNFKEDADYNAALNISNPKLKSTRGEP

SEQ ID NO: 1310 - protein, 726 aa, synthetic construct
SEVEFSHEYWMRHALTLAKRARDEREVPVGAILVLNNRVIGEGWNRAIGLHDPTAHAEIMALRQGGLVLQNYRLIDATLYVTFEPCVMCAGAMIHSRIGRVVFGVRNNKHGAAGSLVNVLNYPGMNHRVEITEGILADECAALLCDFYRMPRLVFNARKKTQSSINPGGSSGGSSSSETPGTSGSATPEGSGGSSGGSAKNTITKTLKLRIVRPYNSAEVEKIVADEKNNREKIALEKNKGKVKEACSKHLKVASYCTTQVERNACLFCKARKLDDKFYQKLRGQFPDAVFWQELGEIFRQLQKQAAEIYNQSLIELYYEIFIKGKGFANASSVEHYLSDVCYTRAAELFKNAAIASGLRGKVKSNFRLKELKNMKSGLPTTKSDNFPIPLVKQKGGQYTGFEISSHNSDFIIKIPFGRWQVKEEIDKYRPWEKFDFEQVRKSPKPISLLLSTQRRKRNKGWSKDVGTEAEIRKVMNGDYQTSYIEVKRGSKIGEKSAWMLNLSIDVPKFDKGVDPSIIGGIDVGVKSPLVCAINNAFSRYSISDNDLFRFNKKVFARRRILLKKNRHKRAGHGTKNKLKPITILTEKSGRFRKKLIERWACEIADFFIKNKVGTVQMENLESMKRKEDSYFNIRLRGFWPYAEMQNKIEFKLKQYGIKIRKVAPNNTSKTCSKCGHLNNYFNFEYRKKNKFPHFKCEKCNFKENADYNAALNICNPKLKGTKEEP

SEQ ID NO: 1311 - protein, 726 aa, synthetic construct
SEVEFSHEYWMRRALTLAKRARDEREVPVGAVLVLNNRVIGVGWNRTTGLHDPTAHAEIMALRQGGLVMRNYRLTDATLYVTFEPCVMCAGAMVHSRIGRVVFGVRNSKRGAAGSLMNVLDYPGMNHCVEITEGILVDECAALLCDFYRMPRQVLNAQKKAQPSISSGGSSGGSSGSETPGASGSVTPKSSGGSSGGSAKNTITKTLKLRIVRPYNSAEVEKIVADEKNNREKIALEKNKGKVKEACSKHLEVAAYCTTQVERNACLFCKARKLDDKFYQKLRGQFPDAVFWQEVGEIFRQLQKQAAEIYNQSLIELYYEIFIRGKGFANASSVEHYLSDVCYTRAAELFKNAAIASGLRGKVKSNFRLKELKNMKSGLPTTKSDNFPIPLVKQKGGQYTGFEISSHNDDFIIKIPFGRWQVKKEIDKYRPWEKFDFEQVRKSPKPISLLLSTQRRKRNEGWSKDEGTEAEIRKVMNGDYQTSYIEVKRGSKTGEKSAWMLNLSINVPKIDKGVDPSIIGGIDVGVKSPLVCAINNAFSRYSISDNDLFRFNKKMFARRRILLRKNRHKRAGHGAKNKLKPISILTGKSERFRKKLIERWACEIADFFIKNKVGTVQMENLEGMKRKEDSYFNIRLRGFWPYAEMQNKIEFKLKQYGIEIRKVAPNNTSKTCSKCGHLNNYFNFEYRKKNKFPHFKCEKCNFKENADYNAALNISNPKLKSTKEEP

SEQ ID NO: 1312 - protein, 726 aa, synthetic construct
SEVEFSHEYWMRHALTLAERARDEREVPVGAVLVLNNRVIGEGWNRTTGLHDPTAHAEIMALRQGGLVMQNHRLVDATLYVTFEPCVMCAGAMIHSRIGRVVFGVRNSKRGAAGSLTNVLNYPGMNHRVEITEGILVGECAALLCDFYRMPRQVFSARKKARSTINTGGSSGGSSGSETPGTSESPTPESSGGNPGGSAKNTITKTLKLRIVRPYNSAEVEKIVADEKNNREKIALEKNKDKVREACSKHLKVAAYCTTQVERNACLFCKARKLDDKFYQKLRGQFPDAVFWQEIGEIFRQLQKQAAEIYNQSLIELYYEIFIKGKGFANASSVEHYLSDVCYTRAAELFKNAAIASGLRGKVKSNFRLKELKNMKSGLPTTKSDNFPIPLVKQKGGQYTGFEISSHNDDFIIKIPFGRWQVKKEIDKYRPWEKFDFEQVRKSPKPISLLLSTQRRKRNKGWSKDEGTEAEIRKVMNGDYQTSYIEVKRGSKTGEKSAWMLNLSIDVPKIDKGVDPCIIGGIDVGVKSPLVCAINNAFSRYSISDNDLFHFNKKMYARRRILLKKNGHKRAGHGAKNKLKPITIMTEKSKRFRKKLIERWACEIADFFVKNKVGTVQMENLESMKRKEDSYFNVRLRGFWPYAEMQNKIEFKLKQYGIVVRKVAPNNTSKTCSKCGHLNNYFNFEYRKKNKFPHFKCEKCNFKESADYNAALNISNPKLKSTKEEP

SEQ ID NO: 1313 - protein, 726 aa, synthetic construct
SEVEFSHEYWMRRALTLAKRARDEREVPVGAVLVLNNRVIGVGWNRAVGLHDPTAHAEIMALRQGGLVMQNYRLIEATLYVTFEPCIMCTGAMIHSRIGRVVFGVRNSKRGAAGSLMNVLNYPGMNHRVEITEGILADECAALLCDYYRMPRRVFNARKKVQSSINSGGSSDGGSSSETPGTIESATPESSGGSSGGSAKNTITKTLKLRIVRPYNSAEVEKIVADEKNNREKIALEKNKDRVKEACSEHLKVAAYCTTQVERSACLFCKARKLDDKFYQKLRSQFPDAVFWQEIGEIFRQLQKQAAEIYNQSLIELYYEILIKGKGFANASSVEHYLSDVCYTRAAELFKNAAIASGLRGKVKSSFRLKELKNMRSGLPTTKSDNFPIPLVKQKGGQYTGFEISSHNDDFIIKIPFGRWQVKKEIDKYRPWEKFDFEQVRKSPKPISLLLSTRRRKRNKGWGKDEGTEAEIRKVMNGDYQTSYIEVKRGSKIGEKSAWMLNLSIDVPKIDKGVDPSIIGGIDVGVKSPLVCAINNVLSRYSISDNDLFHFNKKMFARRRILLKKNGHKRAGHGAKNKLKPITIMTEKSKRFRKKLIERWACEIADFFIKNKVGTVQMENLESMKRKEDSYFNIRLRGFWPYAEMQNKIEFKLKQYGIVVRKVAPNNTSKTCSQCGHLNNYFNFEYRKRNKFPHFKCEKCNFKENADYNAALNISNPKLKSTKGEP

SEQ ID NO: 1314 - protein, 726 aa, synthetic construct
SEVEFSHEYWMRHALTLAKRARDEREVPVGAILVLNNRVIGEGWNRAIGLHDPTAHAEIMALRQGGLVMQNYRLTDATLYVTFEPCVMCAGAMIHSRIGRVVFGVRNNKHGAAGSLVNVLNYPGMNHRVEITEGILADECAALLCDFYRMPRQVFNARKKAQSSINPGGSSGGSSGSETPGTSESATPESSGGSSGSSAKNTITKTLKLRIVRPYNSAEVEKIVADEKNNREKIALEKNKDKVKEACSKHLKVAAYCTTQVERNACLFCKARRLDDKFYQKLRGQFPDAVFWQEIGEIFRQLQKQAAEVYNQSLVELYYEILIKGKGIANASSVEHYLSDVCYTRAAELFKNAAIASGLRNKIKSNFRLKELRNMKSGLPTTKSDNFPIPLVRQKGGQYTGFEISNHDGDFIIKIPFGRWQVKKEINKHRPWEKFDFEQVRKSPKPISLLLSTQRRKRNKGWSKDEGTEAEIRKVMNGDYQTSYIEVKRGSKIGEKSAWMLNLSIDVPKIDKGVDPSIIGGIDVGVKSPLVCAINNALSRYSISDNDLFHFNKKMFARRRILLRKNRHKRAGHGAKNKLKPITIMTEKSGRFRKKLIERWACEIADFFIKNKVGTVQMENLESMKRKEDSYFNIRLRGFWPYAEMQNKIEFKLKQYGIKIRKVAPNNTSKTCSKCGHLNNYFSFEYRKKNKFPHFKCEKCYFKENADYNAALNISNPKLMSTKEEP

SEQ ID NO: 1315 - protein, 726 aa, synthetic construct
SEVEFSHEYWMRHALTLAKRARDEREVPVGAILVLNNRVIGEGWNRAIGLHDPTAHAEIMALRQGGLVMQNYRLIDATLYVTFEPCVMCAGAMIHSRIGRVVFGVRNNKHGAAGSLVNVLNYPGMNHRVEITEGILADECAALLCDFYRMPRQVFSARKKAQSSINPGGSSGGSSGSETPGASESATPESSGGSSGGSAKNTITKTLKLRIVRPYNSAEVEKIVADEKNNREKIALEKNKDKVKEACSKHLKVAAYCTTQVERNACPFCKARRLDDKFYQKLRGQFPDAVFWQEIGEIFRQLQKQAAETYNQSLIELYYEIFIKGKGIANASNVEHYLSDVCYTRAAELFKNAAIASGLRNKIKSNFRLKELRNMKSGLPTTKSDNFPIPLVRQKGGQYTGFEISNHNSDFIIKIPFGRWQAKKEIDKYRPWEKFDFEQVRKSPKPISLLLSTQRRKRNKGWSRDEGTEAEIRKVMNGDYQVSYIEVKRGSKIGEKSAWMLNLSIDVPKIDKGVDPSIIGGIDVGVKSPLVCAINDAFSRYSISDNDLFRFNKKMFARRRILLKKNRHKRAGHGAKNKLKPISILTGKSERFRKKLIERWACEIADFFIKNKVGTVQMENLESMKRKEDSYFNIRLRGFWPYAEMQNKIEFKLKQYGIEIRKVAPNNTSKTCSKCGHLNNYFNFEYRKKNKFPHFRCEKCNFKENADYNAALNISNPKLKSTKEKP

SEQ ID NO: 1316 - protein, 726 aa, synthetic construct
SEVEFSHEYWMRHALSLAKRARDEREVPVGAVLVLNNRIIGEGWNRAIGLHDPTAHAEIMALRQGGLVMQNYRLTDATLYVTFEPCVMCAGAMVHGRIGRVVFGVRNSKRGAAGSLMNVLNYPGVNHCVEITEGILVDECAALLCDFYRMPRQVLNAQKKAQSSISPGGSSGGCSGSEMPGASESVTPKSSGGSSAGSTKNTITKTLKLRIVRPYNSAEVEKIVADEKNSREKVALERNKDKVKEACSKHLKVAAYCTTQVERNACLFCKARRLDDKFYQKLRGQFPDAVFWQEIGEIFRQLQKQAAEVYNQSLVELYYEIFIKGKGIANASSVEHYLSDVCYTRAAELFKNAAIASGLRGKVKSNFRLKELKNMKSGLPTTKSDNFPIPLVKQKGGQYTGFEISSHNDDLIVKIPFGRWQVKKEIDKYRPWEKFDFEQVRKSPKPISLLLSTQRRKRNKGWSKDEGTEAEIRKVMNGDYQTSYIEVKRGSKIGEKSTWMLNLSIDVPKIDKGVDPSIIGGIDVGVKSPLVCAINNAFSRYSISDNDLFHYNKKMFARRRILLKKNRHKRAGHGAKNKLKPISILTEKSKRFRKTLIERWACEIADFFIKNKVGTVQIENLESMKRKEDSYFNIRLRGFWPYAEMQNKIEFKLKQYGIVVRKVAPNNTSKTCSKCGHLNNYFNFEYRKKNKFPHFKCEKCNFKEDADYNAALNISNPKLKSTKEEP

SEQ ID NO: 1317 - protein, 726 aa, synthetic construct
SEVEFSHEYWMRHALTLAKRARDEREVPVGAVLVLNNRVIGEGWNRTTGLHDPTAHAEIMALRQGGLVMQNHRLVDATLYVTFEPCVMCAGAMIHSRIGRVVFGVRNSKRGAAGSLMNVLNYPGMNHRVEITEGILADECAALLCDFYRMPRRVFNAQKKAQSSINSGGSSGGSSGSETPGTSESATPESSGGSSGSSAKNTITKTLKLRIVRPYNSAEVEKIVADEKNNREKIALEENKDKVKEACSRHLKVAAYCTTQVERNACLFCKARRLDDKFYQKLRGQFPDAVFWQEIGEIFRQLQKQAAEVYNQSLVELYYEILIKGKGIANASSVEHYLSDVCYTRAAELFKNAAIASGLRGKVKSNFRLKELKNMKSGLPTTKSDNFPIPLVKQKGGQYTGFEISSHNSDFIIKIPFGRWQVKEEIDKYRPWEKFDFEQVRKSPKPISLLLSTQRRKKNKGWSKDEGTEAEIRRVMNGDYQTSYIEVKRGSKIGEKSAWMLNLSIDVPKIDKGVDPSIIGGIDVGVKSPLVCAINNSSSRYSICDNDLFRFNKKMFARRRILLKKNRHKRAGHGAKNKLKPITILTKKSERFRKKLIERWVCEVADFFIKNKVGTVQMENLESMKRKEDSYFNIRLRGFWPYAEMQNRIELKLKQYGIEIRRVAPNNTSKTCSKCGHLNSYFNFEYRKKNKFPHFKCEKCNFKEDADYNAALNISNPKLKSTKEEP

SEQ ID NO: 1318 - protein, 725 aa, synthetic construct
SEVEFSHEYWMRHALTLAKRARDGREVPVGAVLVLNNRVIGEGWNRAIGLHDPTAHAEIMALRQGGLVMQNYRLTDATLYVTFEPCVMCAGAMIHSRIGRVVFGVRNSKRGAAGSLMNVLNYPGMNHCVEITEGILVDECAALLCDFYRMPRQVLNAQKKAQSSISSGGSSGGSSGSGTPGASESVTPKSSGGSSAGSTKNTITKTLKLRIVRPYNSAEVEKIVADEKNSRERIALEKNKDKVKEACSEHLKVAAYCTTQVERNACLFCKARKLDDRFYQKLRGQFPDAVFWQEISEIFRQLQKQTAEIYNQSLIELYYEIFIKGKGFANASRVEHYLSDVCYARAAKLFKNAAIASGLRGKVKSNFRLKELKNMKSGLPTTKSDNFPIPLVRQKGGQYTGFEISSHNDDFIIKIPFGRWQVKKEIDKYRPWEKFDFEQVRKSPKPISLLLSTQRRKRNRGWSKDEGTEAEIRKVMNGGYQTSYIEVKRGSKIGEKSAWMLNLSIDVPRIDKGVDPSIIGGIDVGVKSPLVCAINNAFSRYSISDNDLFRFNKKMFARRRILLGRNRHKRAGHGVKNKLKPITILTEKSGRFRKKLIERWACEIADFFVKNKVGTVQMENLESMKRKEDSYFNIRLRGFWPYAEMQNKIEFKLKQYGIKVRKVAPNNTSKTCSKCGHLNNYFSFEYRKKNKFPYFKCEKCNFKENADYNAALNISNPQLKSTGEP

SEQ ID NO: 1319 - protein, 726 aa, synthetic construct
SEVEFSHEYWMRHALTLAKRARDEREVPVGAVLVLNNRVIGEGWNRAIGLHDPTAHAEIMALRQGGLVMQNYRLTDATLYVTFEPCVMCAGAMIHSRIGRVVFGVRNNKHGAAGSLVNVLDYPGMNHRVEITEGILADECAALLCDFYRMPRQVFNARKKAQSSISPGGSSGGSSGSETPDASESVTPKSSGGSSGGSAKNTITKTLKLRIVRPYNSAEVEKIVADEKNNREKIALEKNKGKVKEACSKHLEVAAYCTTQVERDACLFCKARKLDDKFYQKLRGQFPDAVFWQELGEIFRQLQKQAAEIYNQSLIELYYEIFIKGKGFANASSVEHYLSDVCYTRAAELFKNAAIASGLRGKVKSNFRLKELKNMKSGLPTTKSDNFPIPLVKQKGGQYTGFEISSHNDDFIIKIPFGRWQVRKEIDKYRPWEKFNFEQVRKSPKPISLLLSTQRRKRNKGWSKDAGTEAEIRKVMNGDYQTSYIEVKRGSKIGEKSAWVLSLSIDVPKIDKGVDPSIIGGIDVGVKSPLVCAINNAFSRYSISDNDLFHFNKKVFARRRILLKKNRHRRAGHGAKNKLKPITILTEKSKRFRKKLIERWACEIADFFIKNKVGTVQMENLESMKRKEDSYFNIRLRGFWPYAEMQNKIEFKLKQYGIKIRKVAPDNTSKTCSKCGHLNNYFNFEYRKKNKFPHFKCEKCNFKEDADYNAALNISNPKLKSTKEEP

SEQ ID NO: 1320 - protein, 726 aa, synthetic construct
SEVEFSHEYWMRHALTLAKRARDEREVPVGAVLVLNNRVIGEGWNRAIGLHDPTAHAEIMALRQGGLVMQNYRLTDATLYVTFEPCVMCAGAMIHSRIGRVVFGVRNSKRGAAGSLMNVLNYPGMNHCVEITEGILVDECAALLCDFYRMPRQVLNAQKKAQSSISSGGSSGGSSGNETPGASESATPKSSSGSSAGSTKNTITKTLKLRIVRPYNSAEVEKIVADEKNNRERIALEKNKDKVKEACSKHLKVAAYCTTQVERNACLFCKARKLDDKFYQKLRGQFPDAVFWQELGEIFRQLQKQAAEIYNQSLIELYYEIFIKGKGFANASSVEHYLSDVCYTRAAELFKNAAIASGLRGKVKSNFRLKELKNMKSGLPSTKSDNFPIPLVKQKGGQYTGFEIRGHNDDLIIKIPFGRWQVKKEIDKYRPWEKFDFEQVRKSPKPISLLLSTQRRRRNKGWSKDEGTEAEIRKVMNGDYQTSYIEVKRGSKIGEKSAWMLNLSIDVPKIDKGVDPGIIGGIDVGVQSPLVCAINNAFSRYSISDNDLFHFNKKMFARRRILLKKNGHKRAGHGAKNKLKPITIMTEKSKRFRKKLIERWACEIADFFIKNKVGTVQMENLESMKRKEDSYFNIRLRGFWPYAEMQNKIEFKLKQYGIEIRRVAPNNTSRTCSKCGHLNDYFNFEYRRKYKFPHFKCEKCNFKEDADYNAALNISNPKLKSTKEEP

SEQ ID NO: 1321 - protein, 726 aa, synthetic construct
SEVEFSHEYWMRHALTLAKRARDEREVPVGAVLVLNNRVIGEGWNRAIGLHDPTAHAEIMALRQGGLVTQNYRLIDATLYVTFEPCVMCAGAMVHSRIGRVVFGVRNSKRGAAGSLMNVLDYPGMGHRVEITEGILADECAALLCDFYCMPRQVFNAQKRAQSSINSGGSSGGSSGSETPGTSESATPKSSGGSSGGSAKNTITKALKLRIVRPYNSAEVEKIVADEKNNRERIALEKNKDKVKEACSKHLKVAVYCTTQVERNACLFCKARKLDDKFYQKLRGQFPDAVFWQEIGEIFRQLQKQAAEIYNQSLIELYYEIFIKGKGFANASSVEHYLSDVCYTRAAELFKNAAIASGLRGKVKSNFRLKELKNMRSGLPTTKSDNFPIPLVKQKGGQYAGFEISSHNDDFIIKIPFGRWQVKKEIDKYRPWEKFDFEQVRKSPKPISLLLSTWRRKRNKGWSKDEGTEAEIRKVMNGDYQTSYIEVKRGSKIGEKSVWMLNLSIDVPKIDKGVDPSIIGGIDVGVKSPLVCAINNAFSRYSISDNDLFHFNKKMFARRRILLKKNRHKRAGHGAKNKLKPISILTEKSKRFRKKLIERWACEIADFFIKNKVGTVQMENLESMKRKEDSYFNIRLRGFWPYAEMQNKIEFKLKQYGIEIRKVAPNNTSKTCGKCGHLNNYFNFEYRKKNKFPHFKCEKCNFKENADYNAALNISNPKLKSTKEEP

SEQ ID NO: 1322 - protein, 726 aa, synthetic construct
SEVEFSHEYWMRHALTLAKRARDEREVPVGAVLVLNNRVIGEGWNRAIGLHDPTAHAEIMALRQGGLVLQNYRLVDATLYVTFEPCVLCAGAMVHSRIGRVVFGARNSKRGAAGSLMNILNYPGMNHRVEITEGILADECAALLCDFYRMPRQVFNAQKKAQSSINSGGSSSGSSGSETPSTCESATPESSGGSSGGSARNTITKTLQLRIVRPYNSAEVEKIVTDEKNNREKIALEKNKDKVKEACSKHLKMASYCTTQVERSACLFCKARKLDDKFYQKLRGQFPDAVFWQELGGIFRQLQKQAAEIYNQSLIELYYEIFIKGKGITNASRVEHYLSDVCYTRAAELFKNAAIASGLRSKVRSNFRLKELKNMKSGLPTTKSDNFPIPLVKQKGGQYTGFEISSHNDDFIIKIPFGRWQVKKEIDKYRPWEKFDFEQVRMSPKPISLLLSTQRRKRNKGWSKDEGTEAEIRKVMNGDYQTSYIEVKRGSKTGEKSAWMLNLSIDVPKIDKGVDPCIIGGIDVGVKSPLVCAINNASSRYSISDNDLFHFNKKMFARRRILLKKNGHKRAGHGTKNKLKPITIMTEKSKRFRKKLIERWACEIADFFIKNKVGTVQMENLESMKRKEDSYFNIRLRGFWPYAEMQNKIEFKLKQYGIEIRKVAPNNTSKTCSKCGHLNNYFNFEYRKKNKFPHFKCEKCNFKENADYNAALNISNPKLKSTKEEP

SEQ ID NO: 1323 - protein, 726 aa, synthetic construct
SEVEFSHEYWMRRALTLAKRARDEREVPVGAVLVLNNRVIGVGWNRAAGLHDPTAHAEIMALRQGGLVMQNYRLVEATLYVTFEPCIMCAGAMIHSRIGRVVFGVRNSKRGAAGSLMNVLNYPGMNHRVEITEGILADECAALLCDFYCMPRQVFNAQKRAQSSINSGGSSGGSSGSETPGTSESATPESSGGSSGGSAKNTTTKTLKLRIVRPYNSAEVEKIVADEKNNREKIALEKNKDKVKEACSKHLKMASYCTTQVERSACLFCKARKLDDKFYQKLRGQFPDAVFWQELGGIFRQLQKQAAEIYNQSLIELYYEIFIKGKGITNASRVEHYLSDVCYTRAAELFKNAAIASGLRSKVRSNFRLKELKNMKSGLPTTKSDNFPIPLVKQKGGQYTGFEISSHNSDFIIKIPFGRWQVKEEIDKYRPWEKFDFEQVRKSPKPISLLLSTQRRKKNKGWSKDEGTEAEIRRVMNGDYQTSYIEVKRGSKIGEKSAWMLNLSIDVPKIDKGVNPSIIGGIDVGVKSPLVCAINNSSSRYSICDNDLFRFNKKMFARRRILLKKNRHKRAGHGAKNKLKPITILTERSKRFRKKLIERWACEIADFFIKNKVGTVQMENLESMKRKEDSYFNIRLRGFWPYAEMQNKIEFKLKQYGIEIRKVAPNNTSRTCSKCGHLNNYFNFEYRKENKFPHFKCEKCNFKEDADYNAALNISNPKLKSTKEEP

SEQ ID NO: 1324 - protein, 726 aa, synthetic construct
SEVEFSHEYWMRHALTLAKRARDEREVPVGAVLVLNNRVIGEGWNRAIGLHDPTAHAEIMALRQGGLVIQNYRLDNATLYVTFEPCVMCAGAMIHSRIGRVAFGVRNSKRGAAGSLMNVLNYPGMNHRVEITEGILAGECAALLCDFYRMPRQVFNAQKKAQSNINSGGSSGGNSGSEAPGTSESPTPESSGGSSGGSAKNTITKTLKLRIVRPYNSTEVEKIVADEKNNREKIALEKNKDKVKEACSKHLKVAAYCTTQVERNACLFCKARKLDDKFYQKLRGQFPDAVFWQEIGEIFRQLQKQAAEIYNQSLIELYYEIFIKGKGFANASSVEHYLSDVCYTRAAELFKNAAIASGLRGKVKSNFRLKELKNMKSGLPTTKSDNFPIPLVKQKGGQYTGFEISSHNDDFVIKIPFGRWQVKEEIDKYRPWEKFDFEQVRRSPKPISLLLSTQRRKRNKGWSKDEGTEAEIRKVMNGDYQTSYIEVKRGSKVGEKSAWMLSLSIDVPKIDKGVDPSIIGGIDVGVKSPLVCAINNAFSRYSIGDNDLFHYNKKMFARRRILLKKNKHKRAGHGARNKLKPITVLTEKSERFRKKLIERWACEIADFFIKNKVGTVQMENLESMKRKEDSYFNIRLRGFWPYAEMQNKIEFKLKQYGIEIRKVAPNNTSKTCSKCGHLNNYFNFEYRKKNKFPHFKCEKCNFKENADYNAALNISNPKLKSTKEEP

SEQ ID NO: 1325 - protein, 726 aa, synthetic construct
SEVEFSHEYWMRHALTLAKRARDEREVPVGAVLVLNNRVIGEGWNRAVGLHDPTAHAEIMALRQGGLVMQNHRLIEATLYVTFEPCIMCAGAMIHSRIGRVVFGVRNSKRGAAGSLMNVLNYPGMNHRVEITEGILADECAALLCDYYRMPRQVFNARKKAQSSINSGGSSDGGSGSETPGTSESATPESSGGSSGGSAKNTITKTLKLRIVRPYNSAEVEKIVADEKNNREKIALEKNKDKVKEACSKHLKMASYCTTQVERNACLFCKARKLDDKFYQKLRGQFPDAVFWQELGGIFRQLQKQAAEIYNQSLIELYYEIFIKGKGITNASRVEHYLSDVCYTRAAELFKNAAIASGLRSKVRSNFRLKELKNMKSGLPTTKSDNFPIPLVKQKGGQYTGFEISSHNSDFIIKIPFGRWQEKEEIDKYRPWEKFDFEQVRKSPKPISLLLSTQRRKKNKGWSKDEGTEAEIRRVMNGDYRTSYIEVKRGGKTGEKSAWVLNLSIDVPKIDKGVDPSIIGGIDVGVKSPLVCAINNAFSRYSISDNDLFRFNKKMFARRRILLKKNRHKRAGHGAKNKLKPISILTGKSERFRKKLIERWACEIADFFIKNKVGTVQMENLESMKKKEDSYFNIRLRGFWPYAEMQNRIEFKLKQYGIEIRKVAPNNTSKTCSKCGHLNNYFNFEYRRKYKFPHFKCEKCNFKEDADYNAALNISNPKLKSTKEEP

SEQ ID NO: 1326 - protein, 726 aa, synthetic construct
SEDEFSHEYWMRHALTLAKRARDEREVPVGAILVLNNRVIGEGWNRAIGLHDPTAHAEIMALRQGGLVMQNYRLIDATLYVTFEPCVMCAGAMIHSRIGRVVFGVRNSKHGAAGSLMNVLNYPGMNHRVEITEGILADECAALLCDFYRMPHQVFSARKKAQSSINPGGSSGGSSGSKTPGTSESATPESSGGSSGSSAKNTITKTLKLRIVRPYNSAEVEKIVADEKNNREKIALEKNKDKVKEACSKHLKVAAYCTTQVERNACLFCKARKLDDKFYQKLRGQFPDAVFWQEIGEVFRQLQKQAAEIYNQSLIELYYEIFIKGKGFANASSVEHYLSDVCYTRAAELFKNAAIASGLRGKVKSNFRLKELKNMKSGLPTTKSDNFPIPLVKQKGGQYTGFEISSHNDDFIIKIPFGRWQVKKEIDKYRPWEKFDFEQVRKSPKPISLLLSTQRRKRNKGWSKDEGTEAEIRKVMNGDYQTSYIEVKRGSKTGEKSAWMLNLSIDVPKIDKGVDPSIIGGIDVGVKSPLVCAINNAFSRYSISDNDLFRFNKKMFARRRILLKKNRHKRAGHGAKNKLKPITILTKKSERFRKKLIERWACEIADFFIKNKVGTVQMENLESMKRKEDSYFNIRLRGFWPYAEMQNKIEFKLKQYGIEIRKVAPNNTSKTCSKCGHLNNYFNFEYRKKNKFPHFKCEKCNFKENADYNAALNISNPKLKSTKEEP

SEQ ID NO: 1327 - protein, 726 aa, synthetic construct
SEVEFSHEYWMRHALTLAKRARDEREVPVGAVLVLNNRVIGVGWNRAIGLHDPTAHAEIMALRQGSLVMQNYRLIDATLYVTFEPCAMCAGAMVHSRIGRVVFGVRNSKRGAAGSLMNVLDYPGMGHRVEITEGILADECAALLCDFYCMPRQVFNAQKRAQSSINSGGSSGGSSGSETPGTSESATPESSGGGSSGSAKNTITKTLQLRIVRPYNSAEVEKIVADEKNNREKIALEKNKDKVKEACSKHLKVASYCTTQVERSACPFCKARKLDDKFYQKLGGQFPDAVFWQELGEIFRQLQKQAAEIYNQSLIELYYEIFIKGRGFANASSVEHYLSDVCYTRAADLFKNAAIASGLRGKVKGNFRLKELKNMKSGLPTTKSDNFPIPLVKQKGGQYTGFEISSHNDDFIIKIPFGRWQMKKEIDRYRPWEKFDFEQVRKSPKPISLLLSTQRRKRNKGWSKDEGTEAEIRKVMNGDYQTSYIEVKRGSKIGEKSAWMLSLSIDVPKIDKGVDPSIIGGIDVGVKSPLVCAINNAFCRYSISDNDLFHFNKKMFARRRILLKKSRHKRAGHGAKNKLKPISILTEKSKRFRKKLIERWACEIADFFIKNKVGTVQMENLESMKRKEDSYFNIRLRGFWPYAEMQDKIEFKLKQYGIEIRKVAPNNTSKTCSRCGHLNNYFNFEYRRKNKFPHFKCEKCNFKENADYNAALNISNPKLKSTREEP

SEQ ID NO: 1328 - protein, 726 aa, synthetic construct
SEVEFSHEYWMRHALTLAKRARDEREVPVGAILVLNNRVIGEGWNRAIGLRDPTAHAEIMALRQGGLEMQNYRLIDATLYVTFEPCVMCAGAMIHSRIGRVVFGVRNNKHGAAGSLVNVLNYPGMNHRVEITEGILADECAALLCDFYRMPRQVFNARKKAQSSINPGGSSGGSSGSETPGNSESATPESSGGSSGGSAKNTITKTLKLRIVRPFNSAEVERIVADEKNNREKIALEKNKDKVKEACSEHLKVAAYCTTQVERSACLFCKARKLDDKFYQKLRGQFPDAVFWQEIGEIFRQLQKQAAEIYNQSLIELYYEIFIKGKGFANASSVEHYLSDVCYTRAAELFKNAAIASGLRGKVKSNFRLKELKNMKSGLPTTKSDNFPIPLVKQKGGQYTGFEISSHNDDFIIKIPFGRWQVKKEIDKYRPWEKFDFEQVRKSPKPISLLLSTQRRKRNKGWSKDEGTEAEIRKVMNGDYQTSYIEVKRGSKIGEKSAWMLNLSIDVPKIDKGVDPSIIGGIDVGVRSPLVCAINNAFSRYSISDNDLFRFNKKMFARRRILLKKNRHKRAGHGAKNKLKPITILTEKSRRFRKKLIERWACEIADFFIKNKVGTVQIESLESMKRKEDSYFNVRLRGFWPYAEMQNKIEFKLKQYGIKIRKVAPNNTSKTCSMCGHLNNYFSFEYRKKNKFPHFKCEKCNFKENADYNAALNISNPKLMSTKEGP

SEQ ID NO: 1329 - protein, 726 aa, synthetic construct
SEVEFSHEYWMRHALTLAKRARDEREVPVGAILVLNNRVIGEGWNRAIGLHDPTAHAEIMALRQGGLVMQNYRLIDATLYVTFEPCVMCAGAMIHSRIGRVVFGVRNNKHGAAGSLVNVLNYPGMNHRVEITEGILADECAALLCDYYRMPRQVFNAQKKAQSTINSGGSSGGSSGSETSGTSGSATPGSSGGSSGGSAKNTITKTLKLRIVRPYNGAEVEKIVADEKNNREKIALEKNKDKVKEACSEHLKVAAYCTTQVERNACLFCKARKLDDKFYQKLRGQFPDAVFWQEIGEIFRQLQKQAAEIYNQSLIELYYEIFIKGKGFANASSVEHYLSDVCYTRAAELFKNAAIASGLRGKVKSNFRLKELKNMKSGLPTTKSDNFPIPLVKQKGGQYTGFEISNHNSDFIIKIPFGRWQVKKEIDKYRPWEKFDFEQVRKSPKPISLLLSTQRRKRNKGWSKDEGTEAEIRKVMNGDYQTSYIEVKRGNKVGEKSAWMLNLSIDVPRIDKGVDPSIIGGIDVGVKSPLVCAINNALSRYSIGDNDLFHFNKKMFARRRILLKKNRHKRAGHGARNKLKPITVLTEKSERFRKKLIERWACEIAYFFIKNKVGTVQMENLESMKRREDSYFNTRLRGFWPYAEMQNKIEFKLKQYGIEVRKVAPNNTSKTCSKCGHLNNYFNFEYRKKNKFPHFRCEKCNFKEDADYNAALNISNPKLKSTKEEP

SEQ ID NO: 1330 - protein, 726 aa, synthetic construct
SEVEFSHEYWMRHALTLAKRARDEREVPVGAVLVLNNRVIGEGWNRAIGLHDPTAHAEIMALRQGGLVMQNYRLTDATLYVTFEPCVMCAGAMIHSRIGRVVFGVRNSKHGAAGSLVNVLNYPGMNHRVEITEGILADECAALLCDFYRMPRQVFNARKKAQSSTNPGGSSGGSSGSETPGTSESATPESSGGSSAGSTKNTITKTLKLRIVRPYNSAEVEKIVADEKNNRERIALEKNKDKVKEACSKHLKVAAYCTTQVERNACLFCKARKLDDKFYQKLRDQFPDAVFWQEIGEIFRQLQRQAAEIYNQSLIELYYEIFIKGKGFANASSVEHYLSDVCYTRAAELFKNAAIASGLRSKVRSNFRLKELKNMKSGLPTTKSDNFPIPLVKQKGGQYTGFEISSHNSDFIIKIPFGRWQVKEEIDKFRPWEKFDFEQVRKSPKPISLLLSTQRRKKNKGWSKDEGTEAEIRRVMNGDYQTSYIEVKRGSKIGEKSAWMLNLSIDVPKIDKGVDPSIIGGIDVGVKSPLVCAINNAFSRYSISDNDLFHFNKKMFARRRILLKKNRRRRAGHGAKNKLKPITILTEKSVRFRKKLIERWACEIADFFIKNKVGTVQMENLESMKRKEDSYFNIRLRGFWPYAEMQSKIEFKLKQYGIEIRRVAPNNTSRTCSKCGHLNNYFDFEYRRKYKFPHFKCEKCNFKEDADYNAALNISNPKLKSTKEEP

SEQ ID NO: 1331 - protein, 726 aa, synthetic construct
SEVEFSHEYWMRHALTLAKRARDEREVPVGAVLVLNNRVIGEGWNRAIGLHDPTAHAEIMALRQGGLVLQNYRLVDATLYVTFEPCVLCAGAMVHSRIGRVVFGARNSKRGAAGSLMNILNYPGMNHRVEITEGILADECAALLCDFYRMPRQVFNAQKKAQSSINSGGSSGGSNGSETPGASESATPKSSGGSSAGSTKNTITKTLKLRIVRPYNSAEVEKIVADEKDNREKIALEKNKDKVKEACSKHLKVAAYCTTQVERNACLFCRARKLDDKFYQKLRGQFPDAVFWQEIGEIFRQLQKQAAEIYNQSLIELYYEIFIKGKGFANASSVEHYLSDVCYTRAAELFKNAAIASGLRGKVKSNFRLKELKNMKSGLPTTKSDNFPIPLVKQKGGQYTGFEISNHNSDFIIKIPFGRWQVKKEINKYRPWEKFDFEQVRKSPKPISLLLSTQRRKRNKGWSKDEGTEAEIRKVMNGDYQTSYIEVKRGSRIGEKSAWMLSLSIDVPKIDRGVDPSIIGGIDVGVKSPLVCAINNGLSRYSISDNDLFHFNKKMFARRRILLKKNRHKRAGHGAMNKLKPITTLTEKSRRFRKKLIERWACEIADFFIKNKVGTVQMESLESMKRREDSYFNVRLRGFWPYAEMQNKIEFKLKQYGIKIRKVAPNNTSKTCSMCGHLNNYFNFEYRRKNKFPHFKCEKCNFKENADYNAALNISNPKLKSTKEEP

SEQ ID NO: 1332 - protein, 726 aa, synthetic construct
SEVEFSHEYWMRHALTLAKRARDEREVPVGAVLVLNNRVIGEGWNRAIGLHDPTAHAEIMALRQGGLAMQNYRLVDATLYVTFEPCVLCAGAMVHSRIGRVVFGVRNSKRGAAGSLMNVLNHPGMNHRVEITEGILADECAALLCDFYRMPRQVFNPRKKAQSSINSGGSSGGSSGSETPGTSESATPKSSGGSSGGSAKNTITKALKLRIVRPYNSAEVEKIVADEKNNRERIALEKNKDKVKEACSKHLKVAAYCTTQVERNACLFCKARKLDDRFYQKLRGQFPDAVFWQEIGEIFRQLQKQAAEIYNQSLIELYYEIFIKGKGFANASSVEHYLSDVCYTRAAELFKNAAIASGLRGKVKSNFRLKELKNMKSGLPTTKSDNFPIPLVKQKGGQYTGFEISSHNDDFIIKIPFGRWQVKEEIDKYRPWEKFDFEQVRKNPKPISLLLSTQRRKRNKGWSKDEGTEAEIRKVMNGDYQTSYIEVKRGSKIGEKSAWMLNLSIDVPKIDKGVDPSIIGGIDVGVKSPLVCAINNACSRYSISDNDLFHFNKKMFARRRILLKRNRHKRAGHGAKNKLKPISILTEKSKRFRKKLIERWACGIADFFIKNKVGTVQMENLESMKRKEDSYFNTRLRGFWPYAEMQNKIEFKLKQYGIEIRKVAPNNTSMTCSKCGHLNNYFNFEYRRKNKFPYFKCEKCNFKENADYNAALNISNPKLKSTKEEP

SEQ ID NO: 1333 - protein, 726 aa, synthetic construct
SEVEFSHEYWMRHALTLARRARDEREVPVGAILVLNNRVIGEGWNRAIGLHDPTAHAEIMALRQGGLVMQSYRLVDATLYVTFEPCVMCAGAMIHSRIGRVVFGVRNSKHGAAGSLMNVLNYPGMNHRVEITGGILADECAALLCDFYRMPRQVFNAQKKARSNINSGGSSGGSSGSETLGTSESATPESSGGSSGGSAKNTITKALQLRIVRPYNSAEVEKIVADEKNNREKIALEKNKDKVKEACSKHLKVAAYCTTQVERNACLFCKARKLDDGFYQKLRGQFPDAVFWQEIGEIFRQLQKQAAEIYNQSLIELYYEIFIKGKGFANASSVEHYLSDVCYTRAAELFKNAAIASGLRGKVKSNFRLKELKNMKSGLPTTKSDNFPIPLVKQKGGQYTGFEISSHNDDFIIKIPFGRWQAKEEIDKYRPWEKFDFEQVRKSPKPISLLLSTQRRKRNKGWSKDEGTEAEIKKVMNGDYQTSYIEVKRGSKIGEKSAWMLNLSIDVPKIDKGVDPSIIGGIDVGVKSPLVCAINNAFSRYSISDNDLFHFNKKMFARRRILLKKNRHKRAGHGAKNKLKPITIMTEKSKRFRKKLIERWACEIADFFIKNKVGTVQMENLRSMKRKEDSYFNIRLRGFWPYAEMQNKIEFKLKQYGIEIRKVAPDNTSKTCSKCGHLNNYFNFEYRKKNKFPHFKCEKCNFKENADYNAALNISNPKLKSTKEEP

SEQ ID NO: 1334 - protein, 726 aa, synthetic construct
SEDEFSHEYWMRHALTLAKRARDGREVPVGAVLVLNNRVIGEGWNRAIGLHDPTAHAEIMALRQGGLVMQNYRLIDATLYVTFEPCVMCAGAMVHSRIGRVVFGVRNSKRGAAGSLMNVLDYPGMGHRVEITEGILADECAALLCDFYCMPRQVFNAQKRAQSSINSGGSSGGSSGSETPGTSKSATPESSGGGSSGSAKSTITKTLQLRIVRPYNSAEVEKIVADEKNNREKIALEKNKDRVKEACSKHLKVASYCTTQVERNACLFCKARKLDDKFYQKLRGQFPDAVFWQELGEIFRQLQKQAAEIYNQSLIELYYEIFIKGKGFANASSVEHYLSDVCYTRAAELFKNAAIASGLRGKVKSNFRLKELKNMKSGLPTTKSDNFPIPLVKQKGGQYTGFEISSHNDDFIIKIPFGRWQVKKEIDKYRPWEKFDFEQVRKSPKPISLLLSTQRRTRNKGWSKDEGTEAEIKRVMNGDYQISYIEVKRGSKIGEKSAWMLNLSVDVPKIDKGVDPSIIGGIDVGVKSPLVCAINNALSRYSISDNDLFHFNKRMFARRRILLRGNRHKRAGHGAKNKLKPITILTEKSERFRKKLIERWACEIANFFIKNKVGTVQMENLEGMKRKEDSYFNIRLRGFWPYAEMQNKIEFKLKQYGIEIRKVAPNNTSKTCSKCGHLNNYFNFEYRKKNKFPHFKCEKCNFKENADYNAALNISNPRLKSTKGEP

SEQ ID NO: 1335 - protein, 726 aa, synthetic construct
SEDEFSHEYWMRHALTLAKRARDGREVPVGAVLVLNNRVIGEGWNRAIGLHDPTAHAEIMALRQGGLVMQNYRLIDATLYVTFEPCVMCAGAMVHSRIGRVVFGVRNSKRGAAGSLMNVLNYPGVNHCVEITEGILVDECAALLCDFYRMPRQVLNAQKKAQSSISSGGSSGGCSGSEMPGASESVTPKSSGGSSAGSTKNTITKTLKLRIVRPYNSAEVEKIVADEKNSREKIALERNKDKVKEACSEHLKVAAYCTTQVERNACLFCKARKLDDRFYQKLRGQFPDAVFWQETGEIFRQLQRQAAEIYNQSLIELYYEIFIKGKGFANASSVEHYLSDVCYTRAAELFKNAAIASGLRGKVKSNFRLKELKNMKSGLPTTKSDNFPIPLVKQKGGQYTGFEISSHNDDFIIKIPFGRWQMKKEIDRYRPWEKFDFEQVRKSPKPISLLLSTQRRKRNKGWSKDEGTEAEIRKVMNGDYQTSYIEVKRGSKIGEKSAWMLSLSIDVPKIDKGVDPSIIGGIDVGVKSPLVCAINNAFRRYSISDNDLFHFNKKMFARRRILLKKSRHKRAGHGAKNKLKPISILTEKSKRFRKKLIERWACEIADFFIKNKVGTVQMENLESMKRKEDSYFNIRLRGFWPYAEMQNKVEFKLKQYGIEVRKVAPNNTSKTCSRCGHLNNYFNFEYRKKNKFPHFKCEKCNFKEDADYNAALNISNPKLKSTKEEP

SEQ ID NO: 1336 - protein, 726 aa, synthetic construct
SEVEFSHEYWMRHALTLAKRARDEREVPVGAVLVLNNRVIGEGWNRAIGLHDPTAHAEIMALRQGGLVMQNHRLVDATLYVTFEPCVLCAGAMVHSRIGHVVFGVRNSKRGAAGSLMNVLNYPGMNHRVEITEGILADECAALLCDFYRMPRQVFNAQKKARSNINSGGSSGSSSGSETPGTSESATPESSGGSSGGSAKNTITKTLKLRIVRPYNSAEVEKIVADEKNNRERIALEKNKDKVKEACSKHLKVAAYCTTQVERNACLFCKARKLDDKFYRKLRGQFPDAVFWQEIGEIFRQLQKQAAEIYNQSLIELYYEIFIKGKGFANASSVEHYLSDVCYTRAAELFKNAAIASGLRGKVKSNFRLKELKNMKSGLPTTKSDNFPIPLVKQKGGQYTGFEISSHNDDFIIKIPFGRWQVKKEINKFRPWEKFDLEQVRKSPKPISLLLSTQRRKRNKGWSRDEGTEAEIRKVMNGDYQTSYIEVKRGSKIGEKSAWMLNLSIDVPKIDKGVDPSITGGIDVGVKSPLVCAINNAFSRYSISDNDLFHFNKKMFARRRILLRKNRHKRAGHGAKNKLKPITILTEKSGRFRRKLIERWACEIADFFIKNKVGTVQMENLESMKRKEDSYFNIRLRGFWPYAEMQNKIELKLKQYGIKVRKVAPNNTSKTCSKCGHLNNHFNFEYRKKNKFPHFKCEKCNFKEDADYNAALNISNPKLKSTKEEP

SEQ ID NO: 1337 - protein, 726 aa, synthetic construct
SEVEFSHEYWMRHALTLAKRARDEREVPVGAVLVQNNRVIGEGWNRAIGLHDPTAHAEIMALRQGGLVMQNYRLTDATLYVTFEPCVMCAGAMIHSRIGRVVFGVRNSKRGAAGSLMNVLNYPGMNHCVEITEGILVDECAALLCDFYRMPRQVLNAQKKAQSSIGPGGSSGGSSGSETPGAGESVTPKGSGGSSAGSTKDTITKTLKLRIVRPYNSAEVEKIVADEKNSREKIALGKYKDKVKEACSEHLKVAAYCTTQVERNACLFCKARKLDDGFYQKLRGQFPDAVFWQEIGEIFRQLQKQAAEIYNQSLIELYYEIFIKGKGFANASSVEHYLSDVCYTRAAELFKNAAIASGLRGKVKSNFRLKELKNMKSGLPTTKSDNFPIPLVKQKGGQYTGFEISNHNSDFIIKIPFGRWQVKKEIDKYRPWEKFDFEQVRKSPKPISLLLSTQRRKRNKGWSKDEGTEAEIRKVMNGDYQTSYIEVKRGSKTGEKSAWMLNLSIDVPKIDKGVDPSIIGGIDVGVKSPLVCAINNAFSRYSISDNDLFRFNKKMFARRRILLKKNRHKRAGHGAKNKLKPISILTGKSERFRKKLIERWACEIADFFIKNKVGTVQMENLESMKRKEDSYFNIRLRGFWPYAEMQNKIEFKLKQYGIEIRKVAPNNTSKTCSKCGHLNNYFNFEYRKKNKFPHFKCEKCNFKENADYNAALNISNPKLKSTKEEP

SEQ ID NO: 1338 - protein, 726 aa, synthetic construct
SEVEFSHEYWMRHALTLAKRARDEREVPVGAVLVLNNRVIGEGWNRAIGLHDPTAHAEIMALRQGGLVMQNYRLIDATLYVTFEPCVMCAGAMIHSRIGRVVFGVRNNKHGAAGSLVNVLNYPGMNHRVEITEGILANECAALLCDFYRMPRQVFNARKKAQSSINPGGSSGGSSGSETPGTSESATPESSGGSSGGSAKNTITKALKLRIVRPYNSAEVEKIVADEKNNREKIALEKNKDKVKEACSKHLKVAAYCTTQVERNACLFCKARRLDDKFYQKLRGQFPDAVFWQEIGEVFRQLQKQAAEIYNQSLVELYYEIFIKGKGIANASSVEHYLSDVCYTRAAELFKNAAIASGLRNKIKSNFRLKELRNMKSGLPTTKSDNFPIPLVRQKGGQYTGFEISNHNGDFIIKIPFGRWQVKKEISKHRPWEKFDFEQVRKSPKPISLLLSTQRRKRNKGWSKDEGTEAEIRKVMNGDYQTSYIEVKRGSKTGEKSAWMLNLSIDVPKIDKGVDPCIIGGIDVGVKSPLVCAINNAFSRYSISDNDLFHFNKKMFARRRILLKENGHKRAGHGAKNKLKPITIMTEKSKRFRKKLIERWACEIADFFIKNKVGTVQMENLESMKRKEDSYFNIRLRGFWPYAEMQNKIEFKLKQYGIVVRKVAPNNTSKTCSKCGHLNNYFNFEYRKKNKFPHFKCEKCNFKENADYNAALNISNPKLKSTKGEP

SEQ ID NO: 1339 - protein, 726 aa, synthetic construct
SEVEFSHEYWMRHALTLAKRARDEREVPVGAVLVLNNRVIGEGWNRAIGLHDPTAHAEIMALRQGGLVMQNYRLTDATLYVTFEPCVMCAGAMIHSRIGRVVFGVRNSKRGAAGSLMNVLNYPGMNHCVEITEGILMDECAALLCDFYRMPRQVLSAQKKAQSSISSGGPSGGSSCSETLGTSESATPESSGGSSGGSAKNTITKTLKLRIVRPYNSAEVEKIVADEKNDREKIALEKNKDKVKEACSEHLKVAAYCTTQVERNACLFCKARKLDGKFYQKLRGQFPDAVFWQEISEIFRQLQKQAAEIYNQSLIELYYEIFIKGKGFANASSVEHYLSDVCYTRAAELFKNAAIASGLRGKVKSNFRLKELKSMKSGLPTTKSDNFPIPLVKQKGGQYTGFEISSHNDDFIIKIPFGRWQVKKEIDKYRPWEKFDFEQVRKSPKPISLLLSTQRRKRNKGWSKDEGTEAEIRKVMNGDYQTSYIEVKRGSKTGEKSAWMLNLSIDVPKIDKGVDPSIIGGIDVGVKSPLVCAINNAFSRYSISDNDLFRFNKKMFARRRILLKKNRHKRAGHGAKNKLKPISILTGKSERFRKKLIERWACEIADFFIKNKVGTVQMENLESMKRKEDSYFNIRLRGFWPYAEMQNKIEFKLKQYGIEIRKVAPNNTSKTCSKCGHLNNYFNFEYRKKNKFPHFKCEKCNFKENADYNAALNISNPMLKSTKEEP

SEQ ID NO: 1340 - protein, 726 aa, synthetic construct
SEVEFSHEYWMRHALTLAKRARDEREVPVGAVLVLNNRVIGEGWNCAIGLHDPTAHAEIMALRQGGLVMQNYRLIDATLYVTFEPCVMCAGAMVHSRIGRVVFGVRNSKRGAAGSLMNVLDYPGMGHRVEITEGILADECAALLCDFYRMPRQVFNAQKRAQSSINSGGSSGGSSGSETPGTSESVTPESSGGGSSGSAKNTITKTLQLRIVRPYNSAEVEKIVADEKNNREKIALEKNKDKVKEACSKHLKVASYCTTQVERNACPFCKARKLDDKFYQKLRGQFPDAVFWQELGEILRQLQKQAAEIYNQSLIELYYEIFIKGRGFANAGSVEHYLSDVCYTRAAELFKNAAIASGLRGKVKSNFRLKELKNMKSGLPTTKSDNFPIPLVKQKGGQYTGFEISSHNDDFIIKIPFGRWQVKKEIDKYRPWEKLDFEQVRKSPKPISLLLSTQRRKRNKGWSKDEGTEAEIRKVMNGDYQTSYIEVKRGSKTGEKSAWMLNLSIDVPKIDKGVDPSIIGGIDVGVKSPLVCAINNAFSRYSISDNDLFRFNKKMFARRRVLLKKNRHKRAGHGAKNKLKPISILTGKSERFRKKLIERWACEIADFFIKNKVGTVQMENLESMKRKEDSYFNIRLRGFWPYAEMQNKIEFKLKQYGIEIRKVAPNNTSKTCSKCGHLNNYFNFEYRKKNKFPHFKCEKCNFKENADYNAALNISNPKLKSTKEGP

SEQ ID NO: 1341 - protein, 726 aa, synthetic construct
SEVEFSHEYWMRHALTLAKRARDEREVPVGAILVLNNRVIGEGWNRAIGLHDPTAHAEIMALRQGGLVMQNYRLTDAILYVTFEPCVMCAGAMVHSRIGRVVFGVRNSKRGAAGSLMNVLNYPDMNHYVEITEGILADECAALLCDFYRMPRQVFNAQKKARSNINSGGSSGGSSGSETLGTSESATPESSGGSSGGSAKNTITKTLKLRIVRPYNSAEVEKIVADEKNNREKIALEKNKDKVKEACSEHLKVAAYCTTQVERNACLFCKARKLDDKFYQKLRGQFPDAVFWQEISEIFRQLQKQAAEIYNQSLIELYYEIFIKGKGFANASSVEHYLSDVCYTRAAELFKNAAIASGLRGKVKSNFRLKELKSMKSGLPTTKSDNFPIPLVKQKGGQYAGFEISSHNDDFIIKIPFGRWQVKKEIDKYRPWEKFDFEQVRKSPKPISLLLSTQRRKRNKGWSKDEGTEAEIRKVMNGDYQTSYIEVKRGSKTGEKSAWMLNLSIDVPKIDKGVDPSIIGGIDVGVKSPLVCAINNAFSRYSISDNDLFRFNKKMFARRRILLKKNRHKRAGHGAKNKLKPISILTGKSERFRKKLIERWACEIADFFIKNKVGTVQMENLESMKRKEDSYFNIRLRGFWPYAEMQNKIEFKLRQYGIEIRKVAPNNTSKICSKCGHLNNYFNFEYRKKNKFPHFKCEKCNFKENADYNAALNISNPKLKSTKEKP

SEQ ID NO: 1342 - protein, 726 aa, synthetic construct
DEVEFSHEYWMRHALTLAKRARDEREVPVGAVLVLNNRVIGEGWNRAIGLHDPTAHAEIMALRQGGLVMQNYRLTDATLYVTFEPCVMCAGAMIHSRVGRVVFGVRNSKRGAAGSLMNVLNYPGMNHCVEITEGILVDECAALLCDFYRMPRQVLNAQKKAQSSISPGGSSGGSSGSETPGTSESATPESSGGSSGGSAKNTITKTLKLRIVRPYNSAEVEKIVADEKNNREKIALEKNKDKVKEACSKHLKVAAYCTTQVERNACLFCKARRLDDKFYQKLRGQFPDAVFWQEIGEIFRQLQKQAAEIYNQSLVELYYEIFIKGRGFANAGSVEHYLSDVCYTRAAELFKNAAIASGLRGKVKSNFRLKELRNMKSGLPTTKSDNFPIPLVKQKGGQYTGFEISSLNDDFIIKIPFGRWQAKKEIDKYRPWEKFDFEQVRKSPKPISLLLSTQRRKRNKGWSKDEGTEAEIWKVMNGDYQTSYIEVKRGSKIGEKSAWMLNLSIDVPKIDKGVDPSIIGGIDVGVKSPLVCAINNALSRYSISDNDLFHFNKKMFARRRILLRKNRHKRAGHGARNKLKPITVLTEKSERFRKKLIERWACEIANFFIKNKVGTVQMENLESMKRREDSYFNIRLRGFWPYAEMQNKIEFKLKQYGIEIRKVAPNNTSKTCSKCGHLNNYFNFEFRKKNKFPHFKCEKCNFKENADYNAALNISNPKLKSTKEEP

SEQ ID NO: 1343 - protein, 726 aa, synthetic construct
SEVEFSHEYWMRHALTLARRARDEREVPVGAILVLNNRVIGEGWNRAIGLHDPTAHAEIMALRQGGLVMQNYRLINATLYVTFEPCVMCAGAMIHSRIGRVVFGVRNSKHGAAGSLMNVLNYPGMNHRVEITEGILADECAALLCDFYRMPRQVFSARKKAQSSINSGDSSGGNSGNKTPGTSESATPESSGGSSGGSAKNTITKTLKLRIVRPYNSAEVEKIVADEKNNREKIALEKNKDKVKEACSKHLKVAAYCTTQVERNACQFCKARKLDDKFYQKLRGQFPDAVFWQEIGEIFRQLQKQAAEIYNQSLIELYYEIFIKGKGFANASSVEHYLSDVCYTRAAELFKNAAIASGLRGKVKSNFRLKELKNMKSGLPTTKSDNFPIPLVKQKGGQYTGFEISSHNDDFIIKIPFGRWQVKKEIDKYRPWEKFDFEQVRKSPKPISLLLSTRRRKRNKGWSKDEGTEAEIRKVMNGDYQTSYIEVKRGSKIGEKSAWMLNLSIDVPKIDKGVDPSIIGGIDVGVKSPLVCAINNAFSRYSISDNDLFRFNKKVFARRRILLKKNRHKRAGHGTKNKLKPITILTEKSGRFRKKLIERWACEIADFFIKNKVGTVQMENLESMKRKEDSYFNIRLRGFWPYAEMQNKIEFKLKQYGIEIRKVAPNNTSKTCSKCGHLNNYFNFEYRRKYKFPHFKCEKCNFKEDADYNAALNISNPKLKSTKEEP

SEQ ID NO: 1344 - protein, 726 aa, synthetic construct
SEVEFSHEYWMRHALTLAKRARDEREVPVGAVLVLNNRVIGEGWNRAIGMHDPTAHAEIMALRQGGLVMQNYRLVDATLYVTFEPCVLCAGAMVHSRIGRVVFGVRNSKRGAAGSLMNVLNYPGMNHRVEVTEGILADECAALLCDFYRMPRQVFNARKKARSNINSGGSSGGSSGSETLGTREGATPESSGGSSGGSAKNTITKTLKLRIVRPYNSAEVEKIVVDEKNNREKVALERNKDKVKEACSEHLKVAAYCTTRVERSACLFCKARKLDDKFYQKLRGQFPDAVFWQELGGIFRQLQKQAAEIYNQSLIELYYEIFIKGKGITNASRVEHYLSDVCYTRAAELFKNAAIASGLRSKVRSNFRLKELKNMKSGLPTTKSDNFPIPLVKQKGGQYTGFEISSHNSDFIIKIPFGRWQVKEEIDKYRPWEKFDFEQVRKSPKPISLLLSTQRRKRNKGWGKDEGTEAEIRKVMNGDYQTSYIEVKRGSKIGEKSAWMLSLSIDVPKIDKGVNPSIIGGIDVGVKSPLVCAINNAFSRYSISDNDLFRFNKKMFARRRILLGKNRHKRAGHGVKNKLKPITILTEKSGRFRRKLIERWACEIADFFVKNKVGTVQMENLESMKRKEDSYFNIRLRGFWPYAEMQNKIEFKLKQYGIKVRKVAPNNTSKTCSKCGHLNNYFSFEYRKKNKFPHFKCEKCNFKENADYNAALNISNPKLKSTKEEP

SEQ ID NO: 1345 - protein, 726 aa, synthetic construct
SEAEFSHEYWMRHALTLAKRARDEREVPVGAVLVLNNRVIGEGWNRAIGLHDPTAHAEIMALRQGGLVMQNYRLADATLYVTFEPCVLCAGAMVHSRIGRVVFGVRNNKRGAAGSLMNILNYPGMNHRVEITEGILADECAALLCDFYRMPRQVFNAQKKARSNINPGGSSGGSSGSETPGTSESATPESSGGSSGGSAKNTITKTLKLRIVRPYNSAEVEKIVADEKNNREKIALEKNKDKVKEACSKHLKVASYCTTQVERNACLFCKARKLDDKFYQQLRGQFPDAVFWQEIGEIFRQLQKQAAEIYNQSLVELYYEIFIKGKGIANASSVEHYLSDVCYTRAAELFKNAAIASGLRNKIKSNFRLKELRNMKSGLPTTKSDNFPIPLVRQKGGQYTGFEISNHNSDFIIKIPFGRWQVKKEIDKYRPWEKFDFAQVRKSPKPISLLLSTQRRKRNKGWSKDEGTEAEIRKVMNGDYQTSYIEVKRGSKIGEKSAWMLSLSIDVPKIDKGVDPSIVGGIDVGVKSPLVCAINNALGRYSISDNDLFHFNKKMFARRRILLRKNRHKRAGHGAKNKLKPITILTEKSRRFRKKLIERWACEIADFFIKNKVGTVQMENLESMKRREDSYFNIRLRGFWPYAEMQNKIEFKLKQYGIEIRRVAPNNTSKTCSKCGHLNNYFNFEYRKKNKFPHFKCGKCNFKENADYNAALNISNPKLKGTKEEP

SEQ ID NO: 1346 - protein, 726 aa, synthetic construct
SEVEFSHEYWMRHALTLAKRARDEREVPVGAILVLNNRVIGEGWNRAIGLHDPTAHAEIMALRQGGLVMQNHRLIDATLYVTFEPCVMCAGAMIHSRIGRVVFGARNSKHGAAGSLVNVLNYPGMNHRVEITEGILADECAALLCDFYRMPRQVFNTRKKAQSSINPSGSSGGSSGSVTPGTSESATPESSGGGFGGSAKNTITKTLKLRIVRPYNSAEVEKIVADEKNNREKIALEKNKDKVKEACSKHLKVAAYCTTQVERNACLFCKARKLDDKFYQKLRGQFPDAVFWQEIGEIFRQLQKQAAEIYNQSLIELYYEIFIKGKGFANASSVEHYLSDVCYTRAAELFKNAAIASGLRGKVKSNFRLKELKNMKSGLPTTKSDNFPIPLVKQKGGQYTGFEISSHNDDFIIKIPFGRWQVKKEIDKYRPWEKFDFEQVRKSPKPISLLLSTQRRKRNKGWSKDEGTEAEIRKVMNGDYQTSYIEVKRGSKIGEKSAWMLNLSIDVPKIDKGVDPSIIGGIDVGVKSPLVCAINNASSRYSISDNDLFRFNKKMFARRRILLKKNRHKRAGHGAKNKLKPISILTGKSERFRKKLIERWACEIADFFIKNKVGTVQMENLESMKRKEDSYFNIRLRGFWPYAEMQNKIEFKLKQYGIEIRKVAPNNTSKTCSKCGHLNNYFSFEYRKKNKFPHFMCVKCNFKENADYNAALNISNPKLKSTKGEP

SEQ ID NO: 1347 - protein, 726 aa, synthetic construct
SEVEFSHEYWMRHALTLAKRARDEREVPVGAVLVLNNRVIGGGWNRAIGLHDPTAHAEIMALRQGGLVMQNCRLVDATLYVTFEPCVMCAGAMIHSRIGRVVFGVRNSKRGAAGSLMNVLNYPGMNHRVEITEGILAGECAALLCDFYRMPRQAFNAQKKAQSTINSGGSSGGSSSSETPGTSGSATPEGSGGSSSGSAKNTITKTLKLRIVRPYNSAEVEKIVADEKNNREKIALEKNKDKVKEACSKHLKVASYCTTQVERNACLFCKARRLDDKFYQKLRGQFPDAVFWQELGEIFRQLQKQAAEVYNQSLIELYYEIFIKGKGFANASSVEHYLSDVCYTRAAELFKNAAIASGLRGKVKSNFRLKELKNMKSGLPTTKSDNFPIPLVKQKGGQYTGFEISSHNDDFIIKIPFGRWQVKKEIDKYRPWEKFDFEQVRKSPKPISLLLSTQRRKRNKGWSKDEGTEAEIRKVMNGDYQTSYIEVKRGSKIGEKSAWMLSLSIDVPKIDKGVDPSIIGGIDVGVKSPLVCAINDAFSRYSISDNDLFHFNKKMFARRRILLKKNRHKRVGHGAKNKRKPISILTEKNERFRKKLIERWACEIADFFIKNKVGTVQMENLESMKRKEDSYFNIRLRGFWPYAEMQNKIEFKLKQYGIEIRKVAPINTSKTCSKCGHLNNYFNFEYRKKNKFPHFKCEKCNFKENADYNAALNISNPKLKSTKEEP

SEQ ID NO: 1348 - protein, 726 aa, synthetic construct
SEVEFSHEYWMRHALTLAKRARDEREVPVGAVLVLNNRVIGEGWNRAIGLHDPTAHAEIMALRQGGLVMQNYRLSDATLYVTFEPCVMCAGAMIHSRIGRVVFGVRNSKRGAAGSLMNVLNYPGMNHCVEITEGILVDECAALLCDFYRMPRQVLSAQKKAQSSVSSGGSPGGSSGSETPGASGSVTPKSSVGSSAGSTKNTITKTLKLRIVRPYNSAEVEKIVADEKNNREKIALEKNRDKVKEACSKHLKVAAYCTTQVERNACLFCKARKLDDKFYQKLRGQFPDAVFWQEVGEIFRQLQKQAAEIYNQSLIELYYEIFIKGQGFANASSVEHYLSDVCYTRAAELFKNAAIASGLRGKVKSNFRLKELKNMKSGLPTTKSDNFPIPLVKQKGGQYTGFEISSHNDDFIIKIPFGRWQVKKEIDKYRPWEKFDFEQVRKSPRPISLLLSTQRRKRNKGWSKDEGTEAEIRKVMNGDYQTSYIEVKRGSKIGEKSAWMLNLSIDVPKIDKGVDPSIIGGIDVGVKSPLVCAINNAFSRYSISDNDLFHFNKKMFARRRILLKKNRHKRAGHGAKNKLKPISILTEKSKRFRKKLIERWACEIADFFIKNKVGTVQMENLESMKRKEDSYFNIRLRGFWPYAEMQDRIEFKLKQYGIEIRRVAPNNTSRTCSKCGHLNNYFNFEYRKTNKFPHFKCEKCNFREDADYNAALNISNPKLKSTKEEP

SEQ ID NO: 1349 - protein, 726 aa, synthetic construct
SEVEFSHEYWMRRALTLAKRARDEREVPVGAVLVLNNRVIGVGWNRAVGLHDPTAHAEIMALRQGGLVMQNYRLIEATLYVTFEPCVMCAGAMIHSRIGRVVFGARNSKRGAAGSLMNVLSNPGMNHRVEITEGILADECAALLCDFYRMPRQVFNAQKKAQSSINSGGSSGGSSGSETPSTSESATPESSGGSSGGSAKSTITKTLQLRIVRPYNSAEVEKIVTDEKNNREKIALEKNKDKVKEACSKHLKMASYCTTQVERNACLFCKARKLDDKFYQKLRGQFPDAVFWQELGGIFRQLQKQAAEIYNQSLIELYYEIFIKGKGITNASRVEHYLSDVCYTRAAELFKNAAIASGLRSKVRSNFRLKELKNMRSGLPTTKSDNFPIPLVKQKGGQYTGFEISSHNSDFIIKIPFGRWQVKEEIDKYRPWEKFDFEQVRKSPKPISLLLSTRRRKRNKGWSKDEGTEAEIRKVMNGDYQTSYIEVKRGSKIGEKSAWMLNLSIDVPKIDKGVDPSIIGGIDVGVKSPLVCAINNAFSRYSIGDNDLFHFNKKMFARRRILLKKNRHRRAGHGARNKLKPITVLTEKSKRFRKKLIERWACEIANFFIKNKVGTVQMENLESMKRKEDSYFNIRLRGFWPYAEMQNKIEFKLKQYGIEIRKVAPNNTSKTCSKCGHLNNYFNFEYRKKNKFPHFKCEKCNFKENADYNAALNISNPKLKSTREEP

SEQ ID NO: 1350 - protein, 726 aa, synthetic construct
SEVEFSHEYWMRHALTLAKRARDGREVPVGAVLVLNNRVIGEGWNRAIGLHDPTAHAEIMALRQGGLVMQNYRLIDATLYVTFEPCVMCAGAMVHSRIGRVVFGVRNGKRGAAGSLMNVLDYPGMGHRVEITEGILADECAALLCDFYRMPRQVFNARKKAQSSISSGGSSGGSSGSETPGASGSVTPKSSGGSSAGSTKDTITKTLKLRIVRPYNSAEVEKVVADEKNNREKIAIEKNKDMVKEACSKHLKVASYCTTQVERNACLFCKARKLDDKFYQKLRGQFPDAVFWQELGGIFRQLQKQAAEIYNQSLIELYYEIFIKGKGITNASRVEHYLSDVCYTRAAELFKNAAIASGLRSKVRSNFRLKELRNMKSGLPTTRSDNFPIPLVRQKGGQYTGFGISNHNSDFIIKIPFGRWQVKKEIDKYRPWEKFDFAQVRKSPKPISLLLSTQRRRRNKGWSNDEGTEAEIRKVMNGDYQTSYIEVKRGSKIGEKSAWMLSLSIDVPKIDKGVDPSIVGGIDVGVKSPLVCAINNALGRFSISDNDLFHFNKKMFARRRILLRKNRHKRAGHGAKNKLKPISILTEKSRRFRKKLIERWACEIADFFIKNKVGTVQMEDLESMKRRGDSYFNIRLRGLWPYAEMQNKIEFKLKQYGIEIRKVAPNNTSKTCSKCGHLNNYFNFEYRKKNKFPHFKCEKCNFKENADYNAALNISNPKLKNTKEEP

SEQ ID NO: 1351 - protein, 726 aa, synthetic construct
SEDEFSHEYWMRHALTLAKRARDGREVPVGAVLVLNNRVIGEGWNRAIGLHDPTAHAEIMALRQGGLVMQNYRLIDATLYVTFEPCVMCAGAMVHSRIGRVVFGVRNSKRGAAGSLMNVLNYPGMGHRVEITEGILADECAALLCDFYCMPRQVFNAQKRAQSSINPSGSSGGSSGSVTPGISESATPESSGGGFGGSAKNTITKTLQLRIVRPYNSAEVEKIVADEKNNREKIALEKNKDKVKEACSKHLKVASYCTTQVERNACLFCKARKLDDKFYQKLRGQFPDAVFWQELGEIFRQLQKQAAEIYNQSLIELYYEIFIKGKGFANASSVEHYLSDVCYTRAAELFKNAAIASGLRGKVKSNFRLKELKNMKSGLPTTKSDNFPIPLVKQKGGQYTGFEISSHNDDFIIKIPFGRWQVKKEIDKYRPWEKFDFEQVRKSPKPISLLLSTRRRKRNKGWSKDEGTEAEIKKVMNGDYQTSYIEVKRGSKIGEKSAWMLNLSIDVPKIDKGVDPSIIGGIDVGVKSPLVCAINNAYSRYSISDNDLFRFNKKMFARRRILLKKNRHKRAGHGAKNKLKPITILTEKSGRFRKKLIERWACEIADFFVKNKVGTVQMENLESMKRREDSYFNIRLRGFWPYAEMQNKIEFKLKQYGIKVRRVAPNNTSKTCSKCGHLNNYFNFEYRKKNKFPHFKCEKCNFREDADYNAALNISNPKLKSTKEEP

SEQ ID NO: 1352 - protein, 726 aa, synthetic construct
SEVEFSHEYWMRHALTLAKRARDEREVPVGAILVLNNRVIGVGWNRAVGLHDPTAHAEIMALRQGGLVMQNYRLVEATLYVTFEPCIMCAGAMIHSRIGRVVFGVRNSKRGAAGSLMNVLNYPGMNHRVEITEGILADECAALLCDYYRMPRQVFNARKKAQSSINSGGSSDGGSGSETPGTSESATPESSGGSSGGSAKNTITKTLKLRIVRPYNSAEVEKIVADEKNNREKIALEKNKDKVKEACSEHLKVAAYCTTQVERSACLFCKARKLDDKFYQKLRGQFPDAVFWQELGEILRQLQKQAAEIYNQSLIELYYEIFIKGRGFANASSVEHYLSDVCYTRAAELFKNAAIASGLRGKVKSNFRLKELKNMKSGLPTTKSDNFPIPLVKQKGGQYTGFEISNHNDDFIIKIPFGRWQVKKEIDKYRPWEKFDFEQVRKSPKPISLLLSTQRRKRNKGWSKDEGTEAEIRKVMNGDYQTSYIEVKRGSKTGEKSAWMLNLSIDVPKIDKGVDPSIIGGIDVGVKSPLVCAIDNAFSRYSISDNDLYHFNKKMFAKRRILLRKNRHKRAGHGARNKLKPITVLTEKSERFRKKLIERWACEIADFFIKNKVGTVQMENLESMKRREDSYFNTRLRGFWPYAEMQNKIEFKLKQYGIEIRKVAPNNTSKTCSRCGHLNNYFNFEYRKKNKFPHFKCEKCNFKENADYNAALNISNPRLKSTKEEP

SEQ ID NO: 1353 - protein, 726 aa, synthetic construct
SEVEFSHEYWMRHALTLAKRARDEREVPVGAILVLNNRVIGEGWNRAIGLHDPTAHAEIMALRQGGLVMQNYRLIDATLYVTFEPCVMCAGAMIHSRIGRVVFGVRNNKHGAAGSLVNVLNYPGMNHRVEITEGILADECAALLCDFYRMPRQVFNARKKAQSSINPGGSSGSSSGSETPGTSESATPESSGGGSSCSAKNTITKTLQLRIVRPYNSAEVEKVVADEKDNREKIALEKNKDKVKEACGKHLKVASYCTTQVERNACLFCKARKLDDEFYQKLRGQFPDAVFWQELGGIFRQLQKQAAEIYNQSLIELYYEIFIKGKGIANASRVEHYLSDVCYTRAAELFKNAAIASGLRSKVRSNFRLKELKNMKSGLPTTRSDNFPIPLVKQKGGQYTGFETSSHNSDFIIKIPFGRWQVKEEIDKYRPWEKFDFEQVRKSPKPISLLLSTQRRKKNKGWSKDEGTEAEIRRVMNGDYQTSYIEVKRGSKIGEKSAWMLNLSIDVPKIDKGVDPSIIGGIDVGVKSPLVCAINSSFSRYSICDNDLFRFNKKMFARRRILLKKNRHKRAGHGAKNKLKPITILTKKSERFRKKLIERWACEIADFFIKNKVGTVQMENLESMKRKEDSYFNIRLRGFWPYAEMQNKIEFKLKQYGIEIRKVAPNNTSKTCSKCGHLNNYFNFEYRKMNKFPHFKCEKCNFKENADYNAALNISNPKLKSTKEEP

SEQ ID NO: 1354 - protein, 726 aa, synthetic construct
SEDEFSHEYWMRHALTLAKRARDEREVPVGAVLVLNNRVIGEGWNRTTGLHDPTAHAEIMALRQGGLVMRNYRLTDATLYVTFEPCVMCAGAMIHSRIGRVVFGVRNSKRGAAGSLMNVLNYPGMNHCVEITEGILVDECAALLCDFYRMPRQVLNAQKKAQSSISPGGSSGGSSGSETPGASESVTPKSSGGSSGGSAKNTITKTLKLRIVRPYNSAEVEKIVADEKDNREKIALEKNKDKVREACSKHLKVASYCTTQVERNACPFCKARKLDDKFYQKLRGQFPDAVFWQELGEIFRQLQKQAAEIYNQSLIELYYEIFIKGKGITNASRVEHYLSDVCYTRAAELFKNAAIASGLRNKIKSNFRLKELRNMKSGLPSTKSDNFPIPLVKQRGGQYTGFEISSHNDDFIIKIPFGRWQAKKEIDKYRPWEKFDFEQVRKSPKPISLLLSTQRRKRNRGWSKDEGTEAEIRKVMNGDYQTSYIEVKRGSKIGEKSAWMLNLSIDVPKIDKGVDPSIIGGIDVGVKSPLVCAINNAFSRYSISDNDLFRFNKKMFARRRILLGKNRHKRAGHGVKNKLKPITILTEKSGRFRKKLIERWACEIADFFVKNKVGTVQMENLESMKRKEDSYFNIRLRGFWPYAEMQNKIEFKLKQYGIKVRKVAPNNTSRTCSKCGHLNNYFSFEYRKKNKFPHFKCEKCNFKENADYNAALNISNPKLKSTKEEP

SEQ ID NO: 1355 - protein, 726 aa, synthetic construct
SEVEFSHEYWMRHALTLAMRARDEREVPVGAVLVLNNRAIGEGWNRAVGLHDPTAHAEIMALRQGGLVMQSYRLTDATLYVTFEPCVMCAGAMIHSRIGRVVFGVRNSKHGAAGSLMNVLNYPGMNHRVEITEGILVDECAALLCDFYRMPRQVFNARKKAQSSINPGGSSGGSSGSETPGTSESATPESSGGSSGSSAKNTITKTLKLRIVRPYNSAEVEKIVADEKNSREKIALEKNKDKVKEACSEHLKVAAYCTTRVERNACLFCKARKLDDRFYQKLRGQFPDAVFWQEIGEIFRQLQKQAAEIYNQSLIELYYEIFIKGKGFANASSVEHYLSDVCYTRAAELFKNAAIASGLRGKVKSNFRLKELKNMKSGLPTTKSDNFPIPLVKQKGGQYTGFEISNHNSDFIIKIPFGRWQVKKEIDKYRPWEKFDFEQVRKSPKPISLLLSTQRRKRNKGWSKDEGTEAEIRKVMNGDYQTSYIEVKRGSKIGEKSAWMLNLSIDVPKIDKGVDPSIIGGIDVGVKSPLVCAINNAFSRYSISDNDLFHFNKKMFARRRILLKKNRHKRAGHGAKNKLKPISILAEKSERFRKKLIEKWACEIADFFIKNKVGTVQMENLESMKRKEDSYFNIRLRGFWPYAEMQNKIEFKLKQYGIEIRKVAPNNTSKTCSKCGHLNNYFNFEYRKKNKFPPFKCEKCNFKENADYNAALNISNPKLKSTKEES

SEQ ID NO: 1356 - protein, 726 aa, synthetic construct
SEVEFSHEYWMRHALTLAKRARDEREVPVGAILVLNNRVIGEGWNRAIGLHDPTAHAEIMALRQGGLVMQNYRLIDATLYVTFEPCVMCAGAMIHSRIGRVVFGVRNNKHGAAGSLVNVLDYPGMNHRVEITEGILADECAALLCDFYRMPRQVFNARKKAQSSISPGGSSGGSSGSEAPGTSESATPESSGGNSGGSAKNTITKTLKLRIVRPYNSAEVEKIVADEKNNREKIALEKNKDKVKEACSKHLKVAAYCTTRVERNACLFCKARKLDDKFYQKLRGQFPDAVFWQEIGEVFRQLQKQAAEIYNQSLIELYYEIFIKGKGFANASSVEHYLSDVCYTRAAELFKNAAIASGLRGKVKSNFRLKELKNMKSGLPTTKSDNFPIPLVKQKGGQYTGFEISSHNDDFIIKIPFGRWQVKKEIDKYRPWEKFDFEQVRKSPKPISLLLSTQRRKRNKGWSKDEGTEAEIRKVMNGDYQTSYIEVKRGSKTGEKSAWMLNLSIDVPKIDKGVDPSIIGGIDVGVKSPLVCAINNAFSRYSISDNDLFRFNKKMFARRRILLKKNRHKRAGHGAKNKLKPISILTGKSERFRKKLIERWACEIANFFIKNKVGTVQMENLESMKRKEDSYFNIRLRGFWPYAEMQNKIEFKLKQYGIEIRRVAPNNTSRTCSKCGHLNNYFNFEYRRKYKFPHFKCEKCNFKEDADYNAALNISNPKLKSTKEEP

SEQ ID NO: 1357 - protein, 726 aa, synthetic construct
SENEFSHEYWMRHALTLAKRARDGREVPVGAVLVLNNRVIGEGWNRAIGLHDPTAHAEIMALRQGGLVMQNYRLIDATLYVTFEPCVMCAGAMVHSRIGRVVFGVRNSKRGAAGSLMNVLNYPGMNHRVEITEGILADECAALLCDFYRMPRQVFNAQKKAQSTINSGGSSGGSSSSETPGTSGSATPKSSGGSSGGSAKNTITKTLKLRIVRPYNSAEVEKIVADEKNNREKIALEKNKGKVKEACSKHLEVAAYCTTQVERNACLFCKARKLDDKFYQKLRGQFPDAVFWQELGEIFRQLQKQAAEIYNQSLIELYYEIFIKGKGFANASSVEHYLSDVCYTRAAELFKNAAIASGLRGKVKSNFRLKELKNMKSGLPTTKSDNFPIPLVKQKGGQYTGFEISSHNDDFIIKIPFGRWQVRKEIDKYRPWEKFNFEQVRKSPKPISLLLSTQRRKRNKGWSKDEGTEAEIRKVMNGDYQTSYIEVKRGSKIGEKSAWMLSLSIDVPKIDKGVDPSIIGGIDVGVKSPLVCAINNAFNRYSISDNNLFHFNKKMFARRRILLKKNRHKRAGHGAKNKLKPISTLTEKSERFRKKLIERWACEIADFFIRNKVGTVQMENLEGMKRKEDSYFNIRLRGFWPYAEMQNKIEFKLKQYGIEVRKVAPNNTSKTCSKCGHLNNYFNFEYRKKNKFPHFKCEKCNFKENADYNAALNISNPKLKSTKEEP

SEQ ID NO: 1358 - protein, 726 aa, synthetic construct
SEVEFSHEYWMRHALTLAKRARDEREVPVGAVLVLNNRVIGEGWNRAIGLHDPTAHAEIMALRQGGLAMQNYRLVDATLYVTFEPCVLCAGAMVHSRIGRVVFGVRNSKRGAAGSLMNVLNHPGMNHRVEITGGILADECAALLCDFYCMPRQVFNAQKRAQSSINSGGSSGGSSGSDTPGTSESATPESSGGGSSGSAKNTITKTLQLRIVRPYNSAEVEKIVADEKNNREKIALEKNKGKVKEACSKHLEVAAYCTTQVERNACLFCKARKLDDKFYQKLRGQFPDAVFWQELGEIFRQLQKQAAEIYNQSLIELYYEIFIKGKGFANAGSVEHYLSDVCYTRAAELFKNAAIASGLRGKVKSNFRLKELKNMKSGLPTTKSDNFPIPLVKQKGGQYTGFEISSHNDDFIIKIPFGRWQVKKEIDKYRPWEKFDFEQVRKSPKPISLLLSTQRRKRNKGWSKDEGTEAEIRKVMNGDYQTSYIEVKRGSKIGEKSAWMLNLSIDVPKIDKGVDPSTTGGIDVGVKSPLVCAISNAFSRYSISDNDLFHFNKKMFARRRILLKKSKHKRAGHGVKNKLKPITILTEKSRRFRKKLIERWACEIADFFIKNKVGTVQMENLESMKRKEDSYFNIRLRGFWPYAEMQNKIEFKLKQYGIEIRKVAPNNTSKTCSKCGHLNNYFNFEYRKKNKFPHFKCEKCNFMENADYNAALNISNPKLKSTKEEP

SEQ ID NO: 1359 - protein, 726 aa, synthetic construct
SEVESSHEYWMRHALTLAKRARDEREVPVGAVLVLNNRVIGEGWNRAIGLHDPTAHAEIMALRQGGLVTQNYRLIDATLYVTFEPCVMCAGAMIHSRIGRVVFGVRNNKHGAAGSLVNVLNYPGMNHRVEITEGILADECAALLCDFYRMPRQVFNARKKAQSSIDTGGSSGGSSGSETPGTSESATPESSGGGSSGSAKNTITKTLQLRIVRPYNSAEVEKIVADEKNNRERIALEKNKDKVKEACSKHLKVASYCTTQVERNACLFCKARKLDDKFYQKLRGQFPDAVFWQELGEIFRQLQKQAAEIYNQSLIELYYEIFIKGKGFANASSVEHYLSGVCYTRAAELFKNAAIASGLRGKVKSNFRLKELKNMKSGLPTTKSDNFPIPLVKQKGGQYTGFEVSSHNDDFIIKIPFGRWQVKKEIDKYRPWEKFDFEQVRKSPKPISLLLSTQRRKRNKGWGKDEGTEAEIRKVMNGDYQTSYIEVKRGSKIGEKSAWMLNLSIDVPKIDKGVDPSIIGGIDVGVKSPLVCAINNALSRYSISDNDLFHFNKKMFARRRILLRKNRHKRAGHGVRNKLKPITVLTEKSERFRKKLIERWACEIANFFIKNKVGTVQMENLESMKRREDSYFNIRLRGFWPYAEMQNKIEFKLKQYGIEIRKVAPNNTSKTCSKCGHLNNYFNFEYRKKNKFPHFKCEKCNFKENADYNAALNISNPKLKSTKEEP

SEQ ID NO: 1360 - protein, 726 aa, synthetic construct
SEVEFSHEYWMRHALTLAKRARDEREVPVGAVLVLNNRVIGEGWNRAIGLHDPTAHAEIMALRQGGLVMQNHRLVDATLYVTFEPCVLCAGAMVHSRIGHVVFGVRNSKRGAAGSLMNVLNYPGMNHRVEITEGILADECAALLCDFYRMPRQVFNAQKKARSNINSGGSSGSSSGSETPGTSESATPESSGGSSGGSAKDTITKTLKLRIVRPYNSAEVEKIVADEKNNREKIALEKNKDKVKEACSKHLKVASYCTTQVERNACLFCKARKLDDKFYQKLRGQFPDAVFWQELGGIFRQLQKQAAEIYNQSLIGLYYEIFIKGKGITNASRVEHYLSDVCYTRAAELFKNAAIASGLRSKVRSNFRLKELKNMKSGLPTTKSDNFPIPLVKQKGGQYTGFEISSHNNDFIIKIPFGRWQVKEEIDKYRPWERFDFEQVRKSPKPISLLLSTQRRKRNKGWSNDEGTEAEIRKVMNGDYRTSYIEVKRGSKIGEKSAWMLNLSIDVPKIDKGVDPSIIGGIDVGVKSPLVCAINNAFSRYSISDNDLFHFNKKMFARRRILLKKNRHKRAGHGTKNKLKPITILTEKSGRFRKKLIERWACEIANFFIKNKVGTVQMENLESMKRKGDSYFNIRLRGFWPYAEMQNKIEFKLKQYGIEIRKVAPNNTSKTCSKCGHLNNYFSFEYRKKNKFPHFKCEKCNFKEDADYNAALNISNPKLKSTKEEP

SEQ ID NO: 1361 - protein, 726 aa, synthetic construct
SEDEFSHEYWMRHALTLAKRARDGREVPVGAVLVLNNRVIGEGWNRAIGLHDPTAHAEIMALRQGGLVMQNYRLIDATLYVTFEPCVMCAGAMVHSRIGRVVFGVRNSKRGAAGSLMNVLDYPGMGHRVEITEGILADECAALLCDFYCMPRQVFNAQKRAQSSISSGGSSGGSSGSGTLGASESVTPKSSVGSSAGSTKNTITKTLKLRIVRPYNSAEVEKIVADEKDNREKIALEKNKDKVKEACSKHLKVAAYCTTQVERNACLFCKARKLDDKFYQKLRGQSPDAVFWQEIGEIFRQLQKQAAEIYNQSLIELYYEIFIKGKGFANASSVEHYLSDVCYTRAAGLFKNAAIASGLRSKVRSNFRLKELKNMKSGLPTTKSDNFPIPLVKQKGGQYTGFEISSHNDDFIIKIPFGRWQVKKEIDKYRPWEKFDFEQVRKSPKPISLLLSTQRRKRNKGWSKDEGTEAEIRKVMNGDYQTSYIEVKRGSKIGEKSAWMLNLSIDVPKIDKGVDPSIIGGIDVGVKSPLVCAINNAFSRYSISDNDLFRFNKKMFARRRILLKKNRHKRAGHGAKNKLKPISILTERSERFRKKLIERWACEIADFFIKNKVGTVQMENLESMKRKEDSYFNIRLRGFWPYAEMQNKIEFKLKQYGIEIRKVAPNNTSKTCSKCGHLNNYFNFEYRKKNKFPHFKCEKCNFKENADYNAALNISNPRLKSTKEEP

SEQ ID NO: 1362 - protein, 726 aa, synthetic construct
SEVEFSHEYWMRHALTLAKRARDEREVPVGAILVLNNRVIGEGWNRAIGLHDPTAHAEIMALRQGGLVMQNYRLIDATLYVTFEPCVMCAGAMIHSRIGRVVFGVRNSKRGAAGSLMNVLNYPGMNHCVAITEGILVDECAALLCDFYRMPRQVLSAQKKVQSSVSPGGSSGGSSGSETPGASESVTPKSSGGSSAGSTKDTITKTLKLRIVRPYNSAEVEKVVADEKNNREKIAMEKNKDKVKEACSKHLKVASYCTTQVERNACLFCKARKLDDKFYQKLRGQFPDAVFWQELGGIFRQLQKQAAEIYNQSLIELYYEIFIKGKGITNASRVEHYLSDVCYTRAAELFKNAAIASGLRSKVRSNFRLKELKNMKSGLPTTKSDNFPIPLVKQKGGQYTGFEISSHNDDFIVKIPFGRWQVKKEIDKYRPWEKFDFEQVRKSPKPISLLLSTQRRKRNKGWSKDEGTEAEIKKVMNGDYQTSYIEVKRGSKIGEKSAWVLNLSIDVPKIDKGVDPSIIGGIDVGVKSPLVCAINNAFSRYSISDNDLFHFNKKMFARRRILLKKSKHKRAGHGAKNKLKPITILTEKSRRFRKKLIERWACEIADFFIKNKVGTVQMENLESMKRKEDSYFNIRLRGFWPYAEMQNKIEFKLKQYGIEIRKVAPNNTSKTCSKCGHLNNYFNFEYRKKNKFPHFKCEKCNFKENADYNAALNISNPKLKSTKEEP

SEQ ID NO: 1363 - protein, 726 aa, synthetic construct
SEVEFSHEYWMRHALTLAKRARDEREVPVGAVLVLNNRVIGEGWNRAIGLYDPTAHAEIMALRQGGLVMQNYRLTDATLYVTFEPCVMCAGAMIHSRIGRVVFGVRNSKRGAAGSLMNVLNYPGMNHCVEITEGILVDECAALLCDFYRMPCQVLNAQKKAQPSISSGGSSGGSSGSETPGASESVTPKSSGGGSAGSTKNTITKTLKLRIVRPYNSAEVEKIVADEKNNREKIALEKNKDKVKEACSKHLKVAAYCTTQVERNACLFCKARKLDDKFYQKLRGQFPDAVFWQEIGEIFRQLQKQAAEIYNQSLIELYYEIFIKGKGFANASSVEHYLSDVCYTRAAELFKNAAIASGLRGKVKSNFRLKELKNMKSGLPTTKSDNFPVPLVKQKGGQYTGFEISSHNDDFIIKIPFGRWQVKEEIDKYRPWEKFDFEQVRKNPKPISLLLSTQRRKRNKGWSKDEGTEAEIRKVMNGDYQTSYIEVKRGSKTGEKSAWMLNLSIDVPKIDKGVDPSIIGGIDVGVKSPLVCAINNAFSRYSVSDNDLFRFNKKMFARRRILLKKNRHKRAGHGAKNKLKPISILTGKSERFRKKLIERWACEIADFFIKNKVGTVQMENLESMKRKEDSYFNTRLRGFWPYAEMQNKIEFKLKQYGIEIRKVAPNNTSKTCSKCGHLNNYFNFEYRKKNKFPHFKCEKCNFKENADYNAALNISNPKLKSTKEEP

SEQ ID NO: 1364 - protein, 726 aa, synthetic construct
SEVEFSHEYWMRHALTLAKRARDGREVPVGAVLVLNNRVIGEGWNRAIGLHDPTAHAEIMALRQGGLVMQNYRLIDATLYVTFEPCVMCAGAMVHSRIGRVVFGVRNSKRGAAGSLMNVLDYPGMGHRVEITEGILADECAALLCDFYCMPRQVFNAQKRAQSSINSGGSSGGSSGSETPGTRESATPESSGGGSGGSAKNTITKTLQLRIVRPYNSAEVEKIVADEKNNREKIALEKNKGKVKEACSKHLKVATYCTTQVERNACLFCRARKLDDKFYQKLRGQFPDAVFWQEIGEIFRQLQKQAAEIYNQSLIELYYEIFIKGKGFANACSVEHYLSDVCYTRAAELFKNAAIASGLRGKVKSNFRLKELKNMKSGLPTTKSDNFPIPLVKQKGGQYTGFEISSHNDDFIIKIPFGRWQVKEEIDKYRPWEKFDFEQVRKSPKPISLLLSTQRRKRNKGWSKDEGTEAEIRKVMNGDYQTSYIEVKRGSKIGEKSAWMLNLSIDVPKIDKGVDPSIIGGIDVGVKSPLVCAINNSSSRYCICDNDLFRFNKKMFARRRILLKKNRHKRAGHGAKNKLRPITILTEKSGRFRKKLIERWACEIANFFIKNKVGTVQMENLEGMKRKEDSYFNIRLRGFWPYAEMQNKIEYKLKQYGIKVRKVAPNNTSKTCSKCGHLNNYFSFEYRKKNKFPHFKCEKCNFKENADYNAALNISNPKLKSTKEEP

SEQ ID NO: 1365 - protein, 726 aa, synthetic construct
SEVEFSHEYWMRHALTLAKRARDEREVPVGAVLVLNNRVIGEGWNRAIGLHDPTAHAEIMALRQGGLVMQNYRLTDATLYVTFEPCVMCAGAMIHSRIGRVVFGVRNSKHGAAGSLVNVLNYPGMNHRVEITEGVLADECAALLCDFYRMPRQVFNARKKAQSSINPGGSSGGSSGSETPGTSESATLENSGGSSGGSAKNTITKTLKLRIVRPYNSAEVEKIVADEKNHREKIALEKNKDKVKEACSKHLKVAAYCTTQVERNACLFCKARRLDDKFYQKLRGQFPDAVFWQEIGEIFRQLQKQAAEIYNQSLVELYYEILIKGKGIANASSVEHYLSDVCYTRAAGLFKNAAIASGLRNKIKSNFRLKELRNMKSGLPTTKSDNFPIPLVKQKGGQYTGFEISNHDGDFIIKIPFGRWQEKKEINKHRPWEKFDFEQVRKSPKPISLLLSTQRRKRNKGWSKDEGTEAEIRKVMNGDYQTSYIEVKRGSKIGEKSAWMLNLSIDVPKIDKGVDPSIIGGIDVGVKSPLVCAINNAFSRYSISDNDLFHFNKKMFARRRILLKKSKHRRAGHGAKNKLKPISILTEKSKRFRKKLIERWACEIADFFIKNKVGTVQMENLESMKRKEDSYFNIRLRGFWPYAEMQNKIEFKLKQYGIEIRKVAPNNTSKTCSKCGHLNNYFNFEYRKKNKFPHFKCEKCNFKENADYNAALNISNPKLKSTKEEP

SEQ ID NO: 1366 - protein, 726 aa, synthetic construct
SEVEFSHEYWMRHALTLAKRARDEREVPVGAVLVLNNRVIGEGWNRAIGLHDPTAHAEIMALRQGGLVMQNYRLINATLYVTFEPCVMCAGAMIHSRIGRVVFGVRNSKHGAAGSLMNVLNYPGMNHRVEITEGILADECAALLCDFYRMPRQVFSARKKAQSSINSGGSSGGNSGNKTPGTSESATPESSGGSSGSSAKNTITKTLQLRIVRPYNSAEVEKIVADEKNNREKIALEKNKDKVKEACSKHLKVAAYCTTQVERNACLFCKARRLDDKFYQKLRGQFPDAVFWQEIGEIFRQLQKQAAETYNQSLIELYYEIFIKGKGIANASNVEHYLSDVCYTRAAELFKNAAIASGLRNKIKSNFRLKELRNMKSGLPTTKSDNFPIPLVKQKGGQYTGFEISNHNNDFIIKIPFGRWQAKKEVDRYRPWEKFDFEQVRKSPKPISLLLSTQRRKRNKGWSKDEGTEAEIKRVMNGDYQISYIEVKRGSKIGEKSAWMLSLSVDVPKIDKGVDPSIIGGIDVGVKSPLVCAINNALSRYSISDNDLFHFNKKMFARRRILLRNNRHKRAGHGAKSKLKPITILTEKGERFRKKLIERWACEIANFFIKNKVGTVQMENLESMKRKEDSYFNVRLRGFWPYAEMQNKIEFKLKQYGIEIRKVAPNNTSKTCSRCGHLNNYFNFEYRRKNKFPHFKCEKCNFKENADYNAALNISNPKLKSTKEEP

SEQ ID NO: 1367 - protein, 726 aa, synthetic construct
SEVEFSHEYWMRHALTLAKRARDEREVPVGAVLVLNNRVIGGGWNRAIGLHDPTAHAEIMALRQGGLVMQNYRLIDATLYVTFEPCVMCAGAMIHSRIGRVVFGVRNSKRGAAGSLMNVLNYPGMDHRVEITGGILADECAALLCDFYRMPRRVFNAQKKAQSSINFGDSSGGSSGSGTPGTSESAAPESSGGSSGGSAKNTITKTLKLRIVRPYNSAEVEKIVADEKNSREKIALEKNKDKVREACSKHLKVAAYCTTQVERNACLFCKARRLDDKFYQKLRGQFPDAVFWQEIGEIFRQLQKQAAEIYNQSLIELYYEIFIKGKGFANASSVEHYLSDVCYTRAAELFKNAAIASGLRGKVKSNFRLKELKNMKSGLPTTKSDNFPIPLVKQKGGQYTGFEISSHNDDFIIKIPFGRWQMKKEIDRYRPWEKFDFEQVRKSPKPISLLLSTQRRKRNKGWSKDEGTEAEIRRVMNGDYQTSYIEVKRGSKIGEKSAWMLSLSIDVPKIDKGVDPSIIGGIDVGVKSPLVCAINNAFCRYSISDNDLFHFNKKMFARRRILLKKSRHKRAGHGAKNKLKPISILTEKSKRFRKKLIERWACEIADFFIKNKVGTVQMENLESMKRKEDSYFNIRLRGFWPYAEMQNKIEFKLKQYGIEIRKVAPNNTSKTCSKCGHLNNYFNFEYRKKNKFPHFKCERCNFKEDADYNAALNISNPGLKGTKEEP

SEQ ID NO: 1368 - protein, 726 aa, synthetic construct
SEVEFSHEYWMRHALTLARRARDEREVPVGAILVLNNRVIGEGWNRAIGLHDPTAHAEIMALRQGGLVMQNYRLTDATLYVTFEPCVMCAGAMIHSRISRVVFGVRNSKHGAAGSLVNVLNYPGMNHRVEITEGILADECAALLCDFYRMPRQVFNAQKKARSNINPGGSSGGSSGSETPGTSESPTPESPGGSSGGSAKNTITKTLKLRIVRPYNSAEVEKIVADEKNNREKIALEKNKDKVKEACSKHLKVAAYCTTQVEGNACLFCRARKLDDKFYQKLRGQFPDAVFWQEIGEIFRQLQKQAAEIYNQSLIELYYEIFIKGKGFANASSVEHYLSDVCYTRAAELFKNAAIASGLRGKVKSNFRLKELKNMKSGLPTTKSDNFPIPLVKQKGGQYTGFEISSHNDDFIIKIPFGRWQVKKEIDKYRPWEKFDFEQVRKSPKPISLLLSTRRRKRNKGWSKDEGTEAEIRKVMNGDYQTSYIEVKRGSKIGEKSAWMLNLSIDVPKIDKGVDPSIIGGIDVGVKSPLVCAINNALSRYSISDNDLFHFNKKMFARRRILLRKNRHKRAGHGAKNKLKPITMMTEKSKRFRKKLIERWACEIADFFIKNKVGTVQMENLESMKRKEDSYFNIRLRGFWPYAEMQDKIEFKLKQYGIVVRKVAPNNTSKTCSKCGHLNHYFNFEYRRKNKFPHFKCEKCTFKEDADYNAALNISNPKLKSTKGEP

SEQ ID NO: 1369 - protein, 726 aa, synthetic construct
SEVEFSHEYWMRHALTLAKRARDEREVPVGAILVLNNRVIGVGWNRAIGLHDPTAHAEIMALRQGGLVMQNYRLIDATLYVTFEPCVMCAGAMIHSRIGRVVFGVRNSKRGAAGSLMNVLNYPGMDHRVEITEGILADECAALLCDFYRMPRQVFNARRKAQSSITSGGSSGGSSGSETPGTSESATPESSGGSSGGSAKNTITKTLKLRIVRPYNSAEVEKIVADEKNNREKIALEKNKDKVKEACSKHLKVASYCTTQVERNACPFCKARKLDDKFYQKLRGQFPDAVFWQEIGEIFRQLQKQAAEIYNQSLVELYYEILIKGKGIANASSVEHYLSDVCYTRAAELFKNAAIASGLRNKIKSNFRLKELKNMKSGLPTTKSDNFPIPLVKQKGGQYTGFEISSHNDDFIIKIPFGRWQVKKEIDKYRPWEKFDFEQVRKSPKPISLLLSTQRRKRNKGWSKDEGTEAEVRKVMNGDYQTSYVEVKRGSKIGEKSAWMLNLSIDVPKIDKGVDPSIIGGIDVGVKSPLVCAINNAFSRYSISDNDLFHYNKRMFARRRILLKKNRHKRAGHGAKNKLKPISVLTEKSGRFRKKLIERWACEIADFFIKNKVGTVQMENLGSMKRKEDSYFNIRLRGFWPYAEMQNKIEFKLKQYGIEIRKVAPDNTSKTCSKCGHLNNYFNFEYRKKNKFPHFKCEKCNFMEDADYNAALNISNPKLKSTKEEP

SEQ ID NO: 1370 - protein, 726 aa, synthetic construct
SEVEFSHEYWMRHALTLAKRARDEREVPVGAVLVLNNRVIGVGWNRAVGLHDPTAHAEIMALRQGGLVMQNYRLIEATLYVTFEPCIMCAGAMIHSRIGRVVFGVRNSKRGAAGSLMNVLNYPGMNHRVEITEGILADECAALLCDYYRMPRQVFNARKKAQSSINSGGSSGGSSGSETPGTSESPTPESSGGSPGGSAKNTITKTLKLRIVRPYNSAEVEKIVADEKNSREKIALEKYKDKVKEACSEHLKVAAYCTTQVERNACLFCKARKLDDKFYQKLRGQFPDAVFWQEIGEIFRQLQKQAAEIYNQSLIELYYEIFIKGKGFANASSVEHYLSDVCYTRAAELFKNAAIASGLRGKVKSNFRLKELKNMKSGLPTTKSDNFPIPLVKQKGGQYTGFEVSSHNDDFIIKIPFGRWQVKKEIDKYRPWEKFDFEQVRKNPKPISLLLSTQRRKRNKGWSKDEGTEAEIRKVMNGDYQTSYIEVKRGNKVGEKSAWMLNLSIDAPKIDKGVDPSIIGGIDVGVKSPLVCAINNALSRYSISDNDLFHYNKKMFARRRILLKKNRHKRAGHGAKNKLRPISILTEKSKRFRKKLIERWACEIADFFIKNKVGTVQMENLESMKRKEDSYFNIRLRGFWPYAEMQNKIEFKLKQYGIEIRKVAPNNTSKTCSKCGHLNSYFDFEYRKKNKFPHFKCEKCNFKENADYNAALNISNPKLKSTKEEP

SEQ ID NO: 1371 - protein, 726 aa, synthetic construct
SEVEFSHEYWMRRALTLAKRARDEREVPVGAVLVLNNRVIGVGWNRAVGLHDPTAHAEIMALRQGGLVMQNYRLIDATLYVTFEPCIMCAGAMIHSRIGRVVFGVRNSKRGAAGSLMNVLNYPGMNHRVEITEGILADECAALLCDFYRMPRQVFNARKRARSNINSGGPSGGSSGSETPGTSESATPESSGGGSSGSAKNTITKTLQLRIVRPYNSAEVEKIVADEKNNREKIALEKNKDKVKEACSKHLKVASYCTTQVERNACPFCKARKLDDKFYQKLRGQFPDAVFWQELGEILRQLQKQAAEIYNQSLIELYYEIFIKGRGFANASSVEHYLSDVCYTRAAELFKNAAIASGLRGKVKSNFRLKELKNMKSGLPTTKSDNFPIPLVKQKGGQYTGFEISSHNDDFIIKIPFGRWQVKEEIDKYRPWEKFDFEQVRKNPKPISLLLSTQRRKRNRGWSKDESTEAEIKKVMNGDYQISYIEVKRGTKIGEKSAWMLNLSVDVPKIDKGVDPSIIGGIDVGVKSPLVCAINNALSRYSISDNDLFRFNKRMFARRRILLKKNGHKRAGHGAKNKLKPITILTEKSGRFRKKLIERWACEIADFFIKNKVGTVQMENLESMKRKEDSYFNIRLRGFWPYAEMQNKIEFKLKQYGIKIRKVAPNNTSKTCSKCGHLNDYFNFEYRKKNKFPHFKCEKCNFKEDADYNAALNISNPKLKSTKEEP

SEQ ID NO: 1372 - protein, 726 aa, synthetic construct
SEVEFSHEYWMRHALTLAKRARDEREVPVGAVLVLNNRVIGEGWNRTTGLHDPTAHAEIMALRQGGLVMQNHRLVDATLYVTFEPCVMCAGAMIHSRIGRVVFGVRNSKRGAAGSLTNVLNYPGMNHRVEITEGILADECAALLCDYYRMPRQVFNARKKAQSSINSGGSSDGGSGSETPGTSESATPESSGGSSGGSAKNTITKTLKLRIVRPYNSAEVEKIVADEKNSREKIALEKNKDKVKEACSKHLRVAAYCTTQVERNACLFCKARKLDDKFYQKLRGQFPDAVFWQEISEIFRQLQKQAAEIYNQSLIELYYEIFIKGKGIANASRVEHYLSNVCYTRAAELFKNAAIASGLRNKIKSNFRLKELRNMKSGLPTTKSDNFPIPLVKQKGGQYTGFEISSHNDDFIIKIPFGRWQVKKEIDKYRPWEKFDFEQVRKSPKPISLLLSTQRRKRNKGWSKDEGTEAEIRKVMNGDYQTSYIEVKRGSKIGEKSAWMLNLSIDVPKIDKGVDPSIIGGIDVGVKSPLVCAINNAFSRYSISDNDLFHYNKKMFARRRILLKKNRHKRAGHGAKNKLKPISILTEKSKRFRKKLIERWACEIADFFIRNKVGTVQIENLESMKRKEDSYFNIRLRGFWPYAEMQNKIEFKLKQYGIEIRKVAPNNTSKTCSKCGHLNSYFNFEYRKKNKFPHFKCEKCNFKENADYNAALNISNPKLKSTKEEP

SEQ ID NO: 1373 - protein, 726 aa, synthetic construct
SEVEFSHEYWMRHALTLAKRARDEREVPVGAILVLNNRVIGEGWNRTIGLHDPTAHAEIMALRQGGLVMQNCRLIDATLYVTFEPCVMCAGAMIHSRIGRVVFGVRNNKHGAAGSLVNVLNYPGMNHRVEITEGILADECAALLCDFYRMPRQVFNARKKAQSNINSGGSSGGSSGSEAPGTSESPTPESSGGSSGGSIKNTITKTLKLRIVRPYNSAEVEKIVADEKNNREKIALEKNKDKVKEACSRHLKVAAYCTTQVERNACLFCKARKLDDKFYRKLRGQFPDAVFWQEIGEIFRQLQKQAAEIYNQSLIELYYEIFIKGKGFANASSVEHYLSDVCYTRAAELFKNAAIASGLRGKVKSNFRLKELKNMRSGLPTTKSDNFPIPLVKQKGGQYTGFEISSHNDDFIIRIPFGRWQVKKEIDKYRPWEKFDFEQVRKSPKPISLLLSTQRRKRNKGWSKDEGTEAEIRKVMNGDYQTSYIEVKRGSKTGEKSAWMLNLSIDVPKIDKGVDPCIIGGIDVGVKSPLVCAINNAFGRYSISDNDLFHFNKKMFARRRILLRKNGHKRAGHGAKNKLKPITIMTEKSKRFRKKLIERWACEIADFFIKNKVGTVQMENLESMKRKEDSYFNIRLRGFWPYAEMQNKIEFKLKQYGIVVRKVAPNNTSKTCSECGHLNNYFNFEYRKKNKFPHFKCEKCNFKENADYNAALNISNPRLKSTKEEP

SEQ ID NO: 1374 - protein, 726 aa, synthetic construct
SEDEFSHEYWMRHALTLAKRARDGREVPVGAVLVLNNRVIGEGWNRAIGLHDPTAHAEIMALRQGGLMMQNYRLIDATLYVTFEPCVMCAGAMVHSRIGRVVFGVRNGKRGAAGSLMNVLDYPGMGHRVEITEGILADECAALLCDFYCMPRQVFNAQKRAQSSINSGGSSGGNSGSETPGTSESATPGSSGGGSSGSAKNTITKTLKLRIVRPYNSAEVEKIVADEKNNREKIALEKNKGKVKEACSKHLEVAAYCTTQVERNACLFCKARKLDDKFYQKLRGQFPDAVFWQELGEIFRQLQKQAAEIYNQSLIELYYEIFIKGKGIANASSVEHYLSDVCYTRAAELFKNAAIASGLRNKIKSNFRLKELKNMRSGLPTTKSDNFPIPLVKQKGGQYAGFEISSHNDDFIIKIPFGRWQVKKEIDKYRPWEKFDFEQVRKSPKPISLLLSTQRRKRNKGWSKDEGTEAEIKKVMNGDYQISYIEVKRGSKIGEKSAWMLSLSIDVPKIDKGVDPRTIGGIDVGVKSPLVCAINNVLSRYSISDNDLFHFNKKMFARRRILLKKNGHKRAGHGAKNKLKPITLMTEKSKRFRKKLIERWACEIADFFIKNKVGTVQMENLESMKRKEDSYFNIRLRGFWPYAEMQNKIEFKLKQYGIVVRKVAPNNTSKTCSQCGHLNNYFNFEYRKKNKFPPFKCEKCNFREDADYNAALNISNPKLKSTKEEP

SEQ ID NO: 1375 - protein, 726 aa, synthetic construct
SEVEFSHEYWMRHALTLAKRARDEREVPVGAVLVLNNRVIGEGWNRAIGLHDPTAHAEIMALRQGGLVMQNYRLSDATLYVTFEPCVMCAGAMIHSRIGRVVFGVRNSKRGAAGSLMNVLNYPGMNHCVEITEGILVDECAALLCDFYRMPRQVLSAQKKAQSSVSSGGSSGGSSGSETPGASGSVTPKSSVGSSAGSTKNTITKTLQLRIVRPYNSAEVEKIVADEKNNRERIALEKNKDKVKEACSKHLKVASYCTTQVERNACPFCKARKLDDKFYQKLRGQFPDAVFWQELGEILRQLQKQAAEIYNQSLIELYYEIFIKGRGFANASSVEHYLSDVCYTRAAELFRNAAIASGLRGKVKSNFRLKELKNMKSGLPTTKSDNFPIPLVKQKGGQYTGFEISSHNDDFIIKIPFGRWQVKKEIDKYRPWEKFDFEQVRKSPKPISLLLSTQRRKRNKGWSKDEGTEAEIRKVMNGDYQTSYIEVKRGSKIGERSAWMLNLSIDVPKIDKGVDPSIIGGIDVGVKSPLVCAINNAFSRYSISDNDLFRFNKKMFARRRILLKKNRHKRAGHGAKNKLKPISILTGKSERFRKKLIERWACEIADFFIKNKVGTVQMENLESMKRREDSYFNIRLRGFWPYAEMQNKIEFKLKQYGIVVRKVAPNNTSKTCSKCGHLNDYFNFEYRKKNKFPHFKCEKCNFKEDADYNAALNISNPKLKGTKEEP

SEQ ID NO: 1376 - protein, 726 aa, synthetic construct
SEVEFSHEYWMRHALTLAKRARDEREVPVGAVLVLNNRVIGEGWNRTTGLHDPTAHAEIMALRQGGLVMRNYRLTDATLYVTFEPCVMCAGAMIHSRIGRVVFGVRNSKRGAAGSLMNVLNYPGMNHCVEITEGILVDECAALLCDFYRMPRQVLNAQKRAQSSISPGGSSGGSSGSETPGASESVTPKSSGGSSGGSAKNTITKTLKLRIVRPYNSAEVEKIVADEKNNREKIALEKNKGKVKEACSKHLEVAAYCTTQVERNACLFCKARKLDDKFYQRLRGQFPDAVFWQELGEIFRQLQRQAAEIYNQSLIELYYEIFIKGKGLANASSVEHYLSDVCYTRAAELFKNAAIASGLRGKVKSNFRLKELKNMKSGLPTTKSDNFPIPLVKQKGGQYTGFEISSHNDDFIIKIPFGRWQVRKEIDKYRPWEKFNFEQVRKSPKPISLLLSTQRRRRNKGWSKDEGTEAEIRKVMNGDYQTSYIEVKRGSKIGEKSAWMLSLSIDVPKIDKGVDPSIIGGIDVGVKSPLVCAINNAFNRYSISDNNLFHFNKKMFARRRILLKKNRHKRAGHGAKNKLRPISILTEKSERFRKKLIERWACEIADFFIRNKVGTVQMENLEGMKRKEDSYFNIRLRGFWPYAEMQNKIEFKLKQYGIEVRKVAPNNTSKTCSKCGHLNNYFNFEFRKKNKFPHFKCEKCNFKENADYNAALNISNPKLKSAKEEP

SEQ ID NO: 1377 - protein, 726 aa, synthetic construct
SEVEFSHEYWMRHALTLAKRARDEREVPVGAVLVLNNRVIGEGWNRAIGLHDPTAHAEIMALRQGGLVMQSYRLSDATLYVTFEPCVMCAGAMIHSRIGRVVFGVRNSKRGAAGSLMNVLNYPGMNHCVEITEGILVDECAALLCDFYRMPRQVLSAQKKAQSSIGSGGSSGGSSGSETPGASGSVTPKSSVGSSAGSTKNTITKTLKLRIVRPYNSAEVEKIVADEKNNREKVALEKNKDKVKEACSKHLKVAAYCTTQVERNACLFCKARKLDDKFYQKLRGQFPDAVFWQEIGEIFRQLQKQAAEIYNQSLIELYYEIFIKGKGFANASSAEHYLSDVCYTRAAELFKNAAIASGLRGKVKSNFRLKELKNMKSGLPTTKSDNFPIPLVKQKGGKYTGFEISSHNDDFIIKIPFGRWQVKKEIDKYRPWEKFDFEQVRKSPKPISLLLSTQRRKRNKGWSKDEGTEAEIRKVMNGDYQTSYIEVKRGSKIGEKSAWMLNLSIDVPKIDKGVDPSIIGGIDVGVKSPLVCAINNSSSRYSICDNDLFRFNKKMFARRRILLKKNRHKRAGHGAKNKLKPITILTKKSERFRKKLIERWVCEVADFFIKNKVGTVQMENLESMKRKEDSYFNIRLRGFWPYAEMQNKIEFKLKQYGIEIRKVAPNNTSKTCSKCGHLNNYFNFEYRKKNKFPHFKCEKCNFKENADYNAALNISNPKLKSTKEEP

SEQ ID NO: 1378 - protein, 726 aa, synthetic construct
SEVEFSHEYWMRHALTLAKRARDEREVPVGAILVLNNRVIGEGWNRAIGLHDPTAHAEIMALRQGGLVMQNYRLIDATLYVTFEPCVMCAGAMIHSRIGRVVFGVRNNKHGAAGSLVNVLNYPGMNHRVEITEGILADECAALLCDFYRMPRQVFNAQKRAQSSINSGGSSGGSSGSETPGTSESATPESSGGGSSGSAKNTITKTLQLRIVRPYNSAEVEKIVADEKNNREKIALEKNKDKVKEACSKHLKVASYCTTQVERNACPFCKARKLDDKFYQKLRGQFPDAVFWQELGEILRQLQKQAAEIYNQSLIELYYEIFIKGGGFANASSVEHYLSDVCYTRAAELFKNAAIASGLRGKVKSNFRLKELKNMKSGLPTTKSDNFPIPLVKQKGGQYTGFEISSHNDDFIIKIPFGRWQVKKEIDKYRPWEKFDFEQVRKSPKPISLLLSTQRRKRNKGWSKDEGTEAEIRKVMNGDYRTSYIEVKRGSKTGEKSAWMLNLSIDVPKIDKGVDPSIIGGIDVGVKSPLVCAINNAFSRYSISDNDLFRFNKKMFARRRILLRKNRHKRAGHGARNKLKPITVLTEKNERFRKKLIERWACEIANFFIKNKVGTVQMENLESMKRREDSYFNIRLRGFWPYAEMQSKIEFKLKQYGIEVRKVAPNNTSKTCSKCGHLNNYFNFEFRKKSKFPHFKCEKCNFKEDADYNAALNISNPKLKSTKEEP

SEQ ID NO: 1379 - protein, 726 aa, synthetic construct
SEDEFSHEYWMRHALTLAKRARDGREVPVGAVLVLNNRVIGEGWNRAIGLHDPTAHAEIMALRQGGLVMQNYRLIDATLYVTFEPCVMCAGAMVHSRIGRVVFGVRNSKRGAAGSLMNVLDYPGMGHRVEITEGILADECAALLCDFYCMPRQVFNAQKRAQSSINSGGSSGGSSGSETPGTSESATPESSGGGSSGSAKNTITKTLQLRIVRPYNSAEVEKIVTDEKNNREKIALEKNKDKVKEACSKHLKMASYCTTQVERNACLFCKARKLDDKFYQKLRGQFPDAVFWQELGGIFRQLQKQAAEIYNQSLIELYYEIFIKGKGITNASRVEHYLSDVCYTRAAELFKNAAIASGLRSKVRSNFRLKELKNMKSGLPTTKSDNFPIPLVKQKGGQYTGFEISSHNDDFIIKIPFGRWQMKKEVDKYRPWEKFDFEQVRKSPKPISLLLSTQRRKRRKGWSKDEGTEAEIRKVMNGDYQTSYVEVKRGSKIGEKSAWMLNLSIDVPKIDKGVDPSIVGGIDVGVKSPLVCAIDNALSRYSISDNDLFHFNKKMFARRRILLKKNRHRRAGHGAKNKLKPISILTEKSKRFRKKLIERWACEIADFFIKNKVGTVQMENLESMKRKEDSYFNIRLRGFWPYAEMQNKIEFKLKQYGIEIRKVAPNNTSKTCSKCGHLNNYFNFEYRKKNKFPHFKCEKCNFKENADYNAALNISNPMLKSTKEEP

SEQ ID NO: 1380 - protein, 726 aa, synthetic construct
SEVEFSHEYWMRHALTLAKRARDEREVPVGAILVLNNRVIGEGWNRAIGLHDPTAHAEIMALRQGGLAMQNYRLIDATLYVTFEPCVMCAGAMIHSRIGRVVFGVRNSKHGAAGSLVNVLNYPGMNHRVEITEGILADECAALLCDFYRMPRQVFNAQKKARSSINSGGSSDGGSGSETPGTSESATPESSGGSSGGSAKNTITKTLKLRIVRPYNSAEVEKIVADEKNNREEIALEKNKDKVKEACSEHLKVAAYCTTQVERSACLFCKARKLDDKFYQKLRGQFPDAVFWQEIGEIFRQLQKQAAEIYNQSLIELYYEIFIKGKGFANASSVEHYLSDVCYTRAAELFKNAAIASGLRGKVKSNFRLKELKNMKSGLPTTKSDNFPIPLVKQKGGQYAGFEISNHNGDFIIKIPFGRWQVKKEVDRYRPWEKFDFEQVRKSPKPISLLLSTQRRKGNKGWSKDEGTEAEIKKVMNGDYQTSYIEVKRGSKIGEKSAWTLNLSIDVPKIDKGVDPSIIGGIDVGVKSPLVCAINNAFSRYSISDNDLFRFNKKMFARRRILLKKNRHKRAGHGAKNKLKPISILTGKSERFRKKLIERWACEIADFFIKNKVGTVQMENLESMKRKEDSYFNIRLRGFWPYAEMQNKIEFKLKQYGIKIRKVAPNNTSRTCSKCGHLNNYFNFEYRRKNKFPHFKCEKCNFKENADYNAALNISNPKLKSTKEEP

SEQ ID NO: 1381 - protein, 726 aa, synthetic construct
SEVEFSHEYWMRHALTLAKRARDEREVPVGAVLVLNNRVIGEGWNRAIGLHDPTAHAEIMALRQGGLVMQNYRLTDATLYVTFEPCVMCAGAMIHSRIGRVVFGVRNSKRGAAGSLMNVLNYPGMNHCVEVTEGILVDECAALLCDFYRMPRQVFNARKKAQSSINPSGSSGGSSGSVTPGTSESATPESSGGSSGGSAKNTITKTLKLRIVRPYNSAEVEKIVADEKNNREKIALEKNKDKVKEACSKHLKVASYCTTQVERSACPFCKARKLDDRFYQKLRGQFPDAVFWQEIGEIFRQLQRQAAEIYNQSLIELYYEIFIKGKGFANASSVEHYLSDVCYTRAAELFKNAAIASGLRGKVKSNFRLKELKNMKSGLPTTKSDNFPIPLVKQKGGKYTGFEISSHNSDFVIKIPFGRWQVKKEIDKYRPWEKFDFEQVRKSPKPISLLLSTQRRRRNKGWSRDEGTEAEIRKVMNGDYQTSYIEVKRGSKIGEKSAWMLNLSIDVPKIDKGVDPSIIGGIDVGVKSPLVCAINNALSRYSISDNDLFHFNKKMFARRRILLKKNRHKRAGHGVKNKLKPISILTEKSKRFRKKLIERWACEIADFFIKNKVGTVQMENLESMKRKEDSYFNIRLRGFWPYAEMQDKIEFKLKQYGIEIRKVAPNNTSKTCSRCGHLNNYFNFEYRRKNKFPHFKCEKCNFKENADYNAALNISNPKLKSTKEEP

SEQ ID NO: 1382 - protein, 726 aa, synthetic construct
SEVEFSHEYWMRHALTLAKRARDEREVPVGAVLVLNNRVIGEGWNRAIGLHDPTAHAEIMALHQGGLVMQNYRLIDATLYVTFEPCVMCAGAMIHSRIGRVVFGARNSKRGAAGSLMNVLSYPGMNHRVEITEGILADECAALLCDFYRMPRRVFNAQKKAQSSINSGGSSGGGSSSDTPSTSESTTPESSGGSSGGPAKNTITKTLKLRIVRPYNSAEVEKIVADEKNNREKTALEKNKDKVKEACSKHLKVAAYCTTQVERNACLFCKARKLDDKFYQRLRGQFPDAVFWQEVGEILRQLQKQAAEIYNQSLIELYYEIFIKGKGFANASSVEHYLSDVCYTRAAELFKNAAIASGLRGKVKSNFRLKELKNMKSGLPTTKSDNFPIPLVKQKGGQYTGFEISNRNSDFIIKIPFGRWQVKKEINKYRPWEKFDFEQVRKSPKPISLLLSTQRRKRNKGWSKDEGTEAEIRKVMNGDYQTSYIEVKRGSRIGEKSAWMLSLSIDVPKIDRGVDPSIIGGIDVGVKSPLVCAINNALSRYSISDNDLFHFNKKMFARRRILLKKNRHRRAGHGARNKLKPITVLTEKSKRFRKKLIERWACEIANFFIKNKVGTVQMENLESMKRKEDSYFNTRLRGIWPYAEMQNKIEFKLKQYGIEIRKVAPNNTSKTCSKCGHLNNYFNFEYRKKNKFPHFKCEKCNFKEDADYNAALNISNPRLKGTKEEP

SEQ ID NO: 1383 - protein, 726 aa, synthetic construct
SEVEFSHEYWMRHALTLAKRARDEREVPVGAILVLNNRVIGEGWNRAIGLHDPTAHAEIMALRQGGLVMQNYRLIDATLYVTFEPCVMCAGAMIHSRIGRVVFGVRNNKHGAAGSLVNVLNYPGMNHRVEITEGILADECAALLCDFYRMPRQVFNAQKKARSNINSGGSSGGSSGSVTPGTSESATPESPGGGFGGSAKNTITKTLQLRIVRPYNSAEVEKVVADEKNNREKIALEKNKDKVKEACSKHLKVASYCTTQVERNACLFCKARKLDDKFYQKLRGQFPNAVFWQELGEIFRQLQKQAAEIYNQSLIELYYEILIKGKGLANASSVEHYLSDVCYTRAAELFKNAAIASGLRGKVKSNFRLKELKNMKSGLPTTKSDNFPIPLVKQKGGQYAGFEISNYNGDFIIKIPFGRWQVKEEIDKFRPWEKFDFEQVRKSPKPISLLLSTQRRKKNKGWSKDEGTEAEIRKVMNGDYQTSYIEVKRGSKIGEKSAWMLNLSIDVPRIDKGVDPSIIGGIDVGVKSPLVCAINNALSRYSISDNDLFHFNKKMFARRRILLRKNRHKRAGHGAKNKLKPITIMTEKSKRFRKKLIERWACEIADFFIKNKVGTVQMENLESMKRKEDSYFNIRLRGFWPYAEMQNKIEFKLKQYGIVVRKVAPNNTSKTCSKCGHLNNHFNFEYRRKNKFPHFKCEECNFKEDADYNAALNISNPKLKSTKGEP

SEQ ID NO: 1384 - protein, 726 aa, synthetic construct; identical to SEQ ID NO: 1112

SEQ ID NO: 1385 - protein, 726 aa, synthetic construct
SEVEFSHEYWMRHALTLAKRARDEREVPVGAVLVLNNRVIGVGWNRAVGLHDPTAHAEIMALRQGGLVTQNYRLVDATLYVTFEPCVMCAGAMIHSRIGRVVFGVRNGKRGAAGSLMNVLNYPGMNHRVEVTEGILADECAALLCDFYRMPRRAFNARKKAQSSTNPGGSSGGSSGSETPGTSESATPESPGGSSGGSAKNTITKTLKLRIVRPYNSAEVEKIVADEKNNREKIALEKNKDKVKEACSKHLKVAAYCTTQVERNACLFCKARRLDDKFYQKLRGQFPDAVFWQEIGEIFRQLQKQAAEIYNQSLIELYYEIFIKGKGFANASSVEHYLSDVCYTRAAELFKNAAIASGLRGKVKSNFRLKELKNMRSGLPTTKSDNFPIPLVKQKGGQYTGFEISSHNDDFIIKIPFGRWQVKKEIDKYRPWEKFDFEQVRKSPKPISLLLSTQRRKRNKGWGKDEGTEAEIRKVMNGDYRTSYIEVKRGSKIGEKSAWMLSLSIDVPKIDKGVDPRIIGGIDVGVKSPLVCAINNAFSRYSISDNDLFHFNKKMFARRRILLKKNRHKRAGHGAKNKLKPITILTEKGVRFRKKLIERWACEIADFFIKNKVGTVQMENLESMKRKEDSYFNIRLRGFWPYAEMQNKIEFKLKQYGIEIRKVAPNNTSKTCSKCGHLNNYFNFEFRKRNKFPHFKCEKCNFKENADYNAALNISNPKLKGTKEEP

SEQ ID NO: 1386 - protein, 726 aa, synthetic construct
SEVEFSHEYWMRHALTLAKRARDEREVPVGAVLVLNNRVIGEGWNRAIGLHDPTAHAEIMALHQGGLVMQNYRLIDATLYVTFEPCVMCAGAMIHSRIGRVVFGARNSKRGAAGSLMNVLSYPGMNHRVEVTEGILADECAALLCDFYRMPRRVFNAQKKAQSSINSVGSSGGGSGSETPSTSESATPESSGGSSGGSAKNTITKTLKLRIVRPYNSAEVEKIVADEKNNREKIALEKNKDKVKEACSKHLKVATYCTTQVERNACPFCKARKLDDKFYQKLRGQFPDAVFWQELGEILRQLQKQAAEVYNQSLIELYYEIFIKGRGFANASSVEHYLSDVCYTRAAELFKNAAIASGLRGKVKSNFRLKELRNMKSGLPTTKSDNFPIPLVKQKGGQYTGFEISSHNDDFIIKIPFGRWQVKKEIDKYRPWEKFDFEQVRKSPKPISLLLSTQRRKRNKGWSKDEGTEAEIRKVMNGDYQTSYIEVKRGSKIGEKSAWMLNLSIDVPKIDKGVDPSIIGGIDVGVKSPLVCAINNAISRYSISDNDLFHFNKKMFARRRILLKKNRHKRAGHGAKNKLKPISILTEKSKRFRKKLIERWACEIADFFIKNKVGAVQMENLESMKRKEDSYFNIRLRGFWPYAEMQNKIEFKLKQYGIEIRKVAPNNTSKTCSKCGHLNNYFNFEYRKMNKFPHFKCEKCNFKENADYNAALNISNPKLKSTKEEP

SEQ ID NO: 1387 - protein, 726 aa, synthetic construct
SEVELSHEYWMRHALTLAKRARDEREVPVGAVLVLNNRVIGEGWNRAIGLHDPTAHAEIMALRQGSLVMQNYRLIDATLYVTFEPCVMCAGAMIHSRIGRVVFGARNSKRGAAGSLMNVLSYPGMNHRVEITEGILADECAALLRDFYRMPRRVFNAQKKAQSSINSGGSSGGGSGSDTPSTSESTTPESSGGSSGGPAKNTITKTLKLRIVRPYNSAEVEKIVADEKNNREKTALEKNKDKVKEACSKHLKVAAYCTTQVERNACLFCKARKLDDKFYQKLRGQFPDAVFWQEVGEIFRQLQKQAAEIYNQSLIELYYEIFIKGEGFANASSVEHYLSDVCYTRAAKLFKNAAIASGLRGKVKSNFRLKELKNMKSGLPTTKSDNFPIPLVRQKGGQYTGFEISSHNDDFIIKIPFGRWQVKEEVDKYRPWEKFDFEQVRRNPKPISLLLSTQRRKRNKGWSKDEGTEAEIRKVMNGDYQTSYIEVKRGSKIGEKSAWMLNLSIDVPKIDKGVDPSITGGIDVGVKSPLVCAINNAFSRYSISDNDLYRFNKKVFARRRILLKKNRHKRAGHGTKNKLKPITILTEKSGRFRKKLIERWACEIANFFIKNKVGTVQMENLESMKRKEDSYFNIRLRGFWPYAEMQNKIEFKLKQYGIKIRKVAPNNTSKTCSKCGHLNNYFSFEYRKKNKFPHFKCEKCNFKEDADYNAALNISNPKLKSTKEEP

SEQ ID NO: 1388 - protein, 726 aa, synthetic construct
SEVEFSHEYWMRHALTLAKRARDEREVPVGAVLVLNNRVIGEGWNRATGQNDPTAHAEIMALRQGGLVMQNHRLIDATLYVTFEPCVMCAGAMIHSRIGRVVIGVRNSRRGAAGSLMNVLNHPGMNHRVEITEGILADECAALLCDFYRMPRQVFNAQEKAQSSTNSGGSSGGSSGSETQGTSESATPGSSGGSSGGSAKNTITKTLKLRIVRPYNSAEVEKIVADEKNNRERIALEKNKDKVKEACSKHLKVAAYCTTQVERNACLFCKARKLDDKFYQKLRGQFPDAVFWQEIGEIFRQLQKQAAEIYNQSLIELYYEILIKGKGFANASSVEHYLSDVCYTRAAELFKNAAIASGLRGKVKSNFRLKELKNMKSGLPTTKSDNFPIPLVKQKGGQYTGFEISSHNDDFIIKIPFGRWQVKKEIDKYRPWEKFDFEQVRKSPKPISLLLSTQRRKRNKGWSKDEGTEAEIRKVMNGDYQTSYIEVKRGSKIGEKSAWMLNLSIDVPKIDKGVDPSIIGGIDVGVKSPLVCAINNALSRYSISDNDLFHFNKKMFARRRILLRKNRHKRAGHGAKNKLKPISILTGKSERFRKKLIERWACEIADFFIKNKVGTVQMENLESMKRKEDSYFNIRLRGFWPYAEMQNKIEFKLKQYGIEIRKVAPNNTSKTCSKCGHLNNYFNFEYRKKNKFPHFKCEKCNFKENADYNAALNISNPKLKSTKEEP

SEQ ID NO: 1389 - protein, 726 aa, synthetic construct
SEVEFSHEYWMRHALTLAKRARDGREVPVGAVLVLNNRVIGEGWNRAIGLHDPTAHAEIMALRQGGLVMQNYRLVDATLYVTFEPCVMCAGAMIHSRIGRVVFGVRNNKRGAAGSLMNVLNYPGMNHRVEITEGILADECAVLLCDFYRMPRQVLNAQRKARSCINSGGSSGGSSGSETPGTSESATPESSGGSSGGSAKNTITKTLKLRIVRPYNSAEVEKIVADEKDNRERIALEKNKGKVKEACGKHLKVAAYCTTQVERNACLFCKARKLDDKFYQELRSQFPDAVFWQEIGEIFRQLQKQAAEIYNQSLIELYYEIFIKGKGIANASSVGHYLSDVCYTRAAELFKNAAIASGLRSKIKSNFRLKELRNMRGGLPTTKSDNFPIPLVKQKGGQYTGFEISSHNDDFIIKIPFGRWLVKKEIDKYRPWEKFDFEQVRKSPKPISLLLSTQRRKRNKGWSNDEGTEAEIRKVMNGDYQTSYIEVKRGSKIGEKSAWMLNLSIDVPKIDKGVDPSIVGGIDVGVKSPLVCAIDNALSRYSISDNDLFHFNKKMFARRRVLLKKNRHRRAGHGAKNKLKPISILTEKSKRFRKKLIERWACEIADFFIKNKVGTVQMENLESMKRKEDSYFNIRLRGFWPYAEMQNKIEFKLKQYGIEVRKVAPNNTSKTCSKCGHLNDYFNFEYRKKNKFPHFKCEKCNFKENADYNAALNISNPKLKSTKEEP

SEQ ID NO: 1390 - protein, 726 aa, synthetic construct
GEDEFSHEYWMRHALTLAKRARDGREVPVGAVLVLNNRVIGEGWNRAIGLHDPTAHAEIMALRQGGLVMQNYRLIGATLYVTFEPCVMCAGAMVHSRIGRVVFGVRNSKRGAAGSLMNVLDYPGMGHRVEITEGILADECAALLCDFYCMPRQVFNAQKRAQSSINSGGSSGGSSGSETPGTSESATPESSGGGSSGSAKNTITKTLQLRIVRPYNSAEVEKVVADEKNNREKIALEKNKDKVKEACSKHLKVASYCTTQVERSACPFCKARKLDDKFYQKLGGQFPDAVFWQELGEILRQLQKQAAEIYNQSLIELYYEIFIKGRGFANASSVEHYLSDVCYTRAAELFKNAAIASGLRGKVKSNFRLKELKNMKSGLPTTKSDNFPIPLVKQKGGQYTGFEISSHNDDFIIKIPFGRWQVKKEIDKYRPWEKFDFEQVRKSPKPISLLLSTQRRKRNKGWSKDEGTEAEIRKVMNGDYQISYIEVKRGSKTGEKSAWMLNLSIDVPKIDKGVDPSIIGGIDVGVKSPLVCAINNALSRYSISDNDLFRFNKKMFARRRILLKKNGHKRAGHGAKNKLKPITIMTEKGKRFRKKLIERWACEIADFFIKNKVGTVQMENLESMKRKEDSYFNIRLRGFWPYAEMQNKIEFKLKQYGIVVRKVAPNNTSKTCSKCGHLNNYFNFEYRKKNKFPHFKCEKCNFKENADYNAALNISNPKLKSTKEEP

SEQ ID NO: 1391 - protein, 726 aa, synthetic construct; identical to SEQ ID NO: 684

SEQ ID NO: 1392 - protein, 726 aa, synthetic construct
SEVEFSHEYWMRRALTLAKRARDEREVPVGAVLVLNNRVIGVGWNRAVGLHDPTAHAEIMALRQGGLVMQNYRLIEATLYVTFEPCIMCAGAMIHSRIGRVVFGVRNSKRGAAGSLMNVLNYPGMNHRVEITEGVLADECAALLCDYYRMPRQVFNARKKAQSSINSGGSSDGGSGSETPGTSESATPESSGGSSGGSAKNTITKTLKLRIVRPYNSAEVEKIVADEKNNREKIALEKNKDKVKEACSEHLKVAAYCTTQVERNACLFCRARKLDDKFYQKLRGQFPDAVFWQEIGEIFRQLQKQAAEIYNQSLIELYYEIFIKGKGFANASSVEHYLSDVCYTRAAELFKNAAIASGLRGKVKSNLRLKELKNMKSGLPTTKSDNFPIPLVKQKGGQYTGFEISSHNDDFIIKIPFGRWQVKKEIDKYRPWEKFDFEQVRKSPKPISLLLSTQRRRRNKGWGKDEGTEAEIRKVMNGDYQTSYIEVKRGSKIGEKSAWMLSLSIDVPKIDKGVDPRIIGGIDVGVKSPLVCAINNAFSRYSISDNDLFHFNKKMFARRRILLKKNRHKRAGHGAKNKLKPISILTGKSERFRKKLIERWACEIADFFIKNRVGTVQMENLESMKRKEDSYFNIRLRGFWPYAEMQNKIEFKLKQYGIGIRKVAPNNTSKTCSKCGHLNNYFNFEYRKKNKFPHFKCEKCNFKENADYNAALNISNPKLKSTKEEP

SEQ ID NO: 1393 - protein, 726 aa, synthetic construct
SEVEFSHEYWMRHALTLAKRARDEREVPVGAVLVLNNRVIGEGWNRAIGLHDPTAHAEIMALRQGGLVMQNYRLADATLYVTFEPCVLCAGAMVHSRIGRVVFGVRNSKRGAAGSLMNVLNYPGMNHRVEITEGILADECAALLCDFYRMPRQVFNARKKARSNINSSGSSGGSSGGETPGTSESATPESSGGSSGGSAKNTITKTLKLRIVRPYNSAEVEKIVADEKNNREKIALERNKDKVKEACSEHLKVAAYCTTQVERNACLFCKARKLDDKFYQKLRGQFPDAVFWQELGEIFRQLQKQAAEIYNQSLIELYYEILIKGKGIANASSVEHYLSNVCYTRAAELFKNAAIASGLRNKIKSNFRLKELRNMKSGLPTTKSDNFPIPLVKQKGGQYTGFEISSHNDDFIIKVPFGRWQVKKEIDKYRPWEKFDFEQVRKSPKPISLLLSTQRRKRNKGWSKDVGTEAEIRKVMNGDYQTSYIEVKRGSKIGEKSAWMLNLSIDVPKIDKGVDPSIIGGIDVGVKSPLVCAINNAFSRYSISDNDLFRFNKKMFARRRILLKKNRHQRAGHGAKNKLKPISILTGKSERFRKKLIERWACEIADFFIKNKVGTVQMENLESMKRKEDSYFNTRLRGFWPYAEMQNKIEFKLKQYGIEIRKVAPNNTSKTCSKCGHLNNYFNFEYRRKNKFPHFKCEKCNFKENADYNAALNISNPKLKSTKEEP

SEQ ID NO: 1394 - protein, 725 aa, synthetic construct
SEVEFSHEYWMRHALTLAKRARDEREVPVGAVLVLNNRVIGEGWNRAIGLHDPTAHAEIMALRQGGLVMQNYRLIDATLYVTFEPCVMCAGAMIHSRIGRVVFGVRNSKRGAAGSLMNVLNYPGMNHCVEITEGILVDECAALLCDYYRMPRQVFNARKKAQSSINPGGSSDGGSGSETPGTSESATPGSSGGGSSGSAKNTITKTLQLRIVRPYNSAEVEKIVADEKNNRERIALEKNKDKVKEACSKHLKVAPYCTTQVERNACPFCKARKLDDKFYQKLRGQFPDAVFWQELGEILRQLQKQAAEIYNQSLIELYYEIFIKGRGFANASSVEHYLSDVCYTRAAELFKNAAIASGLRGKVKSNFRLKELKNMKSGLPTTKSDNFPIPLVKQKGGQYTGFEISSHNDDFIIKIPFGRWQVKKEIDKYRPWEKFDFEQVRKSPKPISLLLSTQRRKRNKGWGKDEGTEAEIRKVMDGDYQTSYIEVKRGSKIGEKSAWMLNLSIDVPKIDKGVDPSIIGGIDVGVKSPLVCAINNAFSRYSISDNELFHFNKKMFARRRILLKKSRHKRAGHGAKNKLKPISILTEKSKRFRKKLIERWACEIANFFIKNKVGTVQMENLESMKRREDSYFNIRLRGFWPYAEMQSKIEFKLKQYGIEIRKVAPNNTSKTCSKCGHLNNYFNFEFRKKNKFPHFKCEKCNFKEDADYNAALNISNPKLSTKEEP

SEQ ID NO: 1395 - protein, 726 aa, synthetic construct
SEVEFSHEYWMRHALTLAKRARDEREVPVGAVLVLNNRVIGEGWNRAIGLHDPTAHAEIMALRQGGLVMQNYRLIDATLYVTFEPCVMCAGAMVHSRIGRVVFGVRNSKRGAAGSLMNVLDYPGMGHRVEITEGILVDECAALLCDFYRMPRQVLNAQKKAQSSISSGGSSGGSSCSETPGASESVTPKSSGGSSAGSTKNTITKTLKLRIVRPYNSAEVEKIVADEKNSREKIALEKNKDKVKEACSKHLKVAAYCTTQVERNACLFCKARKLDDKFYQKLRGQFPDAVFWQEIGEIFRQLQKQAAEIYNQSLIELYYEIFIKGRGFANASSVEHYLSDVCYTRAAELFKNAAIASGLRGKVKSNFRLKELKNMKSGLPTTKSDNFPIPLVKQKGGQYTGFEISSHNDDFIIKIPFGRWQVKKEIDKYRPWEKFDFEQVRKSPKPISLLLSTQRRKRNKGWSKDEGTEAEIRKVMNGDYQTSYIEVKRGSKTGEKSAWMLNLSIDVPKVDKGVDPSIIGGIDVGVKSPLVCAINNAFSRYSISDNDLFRFNKKMFARRRILLGKNRHKRAGHGAKNKLKPISILTGKSERFRKKLIERWACEIADFFIKNKVGTVQMENLESMKRKEDSYFNIRLRGFWPYAEMQNKIEFKLKQYGIEIRKVAPNNTSKTCSKCGHLNNYFSFEYRKKNKFPHFKCERCNFKENADYNAALNISNPKLKSTKEEP

SEQ ID NO: 1396 - protein, 726 aa, synthetic construct
SEVEFSHEYWMRHALSLAKRARDEREVPVGAILVLNNRVIGEGWNRAIGLHDPTAHAEIMALRQGGLVMQNYRLIDATLYVTFEPCVMCAGAMIHSRIGRVVFGVRNNKHGAAGSLVNVLNYPGMNHRVEITEGILADECAALLCDFYRMPRQVFNARKKAQSSTNPGGSSGGSSGSEMPGTSESATPESSGGSSGGSAKNTITKTLKLRIVRPYNSAEVEKIVADEKNNREKIALEKNKGKVKEACSKHLKVAAYCTTQVERNACQFCKARKLDDKFYQKLRGQFPDAVFWQELGEILRQLQKQAAEIYNQSLIELYYEIFIKGRGFANASSVEHYLSDVCYTRAAELFKNAAIASGLRGKVKSNFRLKELKNMKSGLPTTKSDNFPIPLVKQKGGQYTGFEISSHNDDFIIKIPFGRWQAKKEIDKYRPWEKFDFEQVRKSPKPISLLLSTQRRKRNRGWSRDEGTEAEIRKVMNGDYQTSYIEVKRGSKTGEKSAWMLNLSIDVPKIDKGVDPSIIGGIDVGVKSPLVCAINNAFSRYSISDNDLFRFNKKMFARRRILLKKNRHKRAGHGTKNKLKPITILTEKSGRFRKKLIERWACEIADFFIKNKVGTVQMENLESMKRKEDSYFNIRLRGFWPYAEMQNKIEFKLKQYGIEIRKVAPNNTSKTCSKCGHLNNYFNFEYRKKNKFPHFKCEKCNFKENADYNAALNISNPKLKSTTEEP

SEQ ID NO: 1397 - protein, 726 aa, synthetic construct
SEVEFSHEYWMRHALTLAKRARDEREVPVGAVLVLNNRVIGGGWNRAIGLHDPTAHAEIMALRQGGLVMQNYRLIDATLYVTFEPCVMCAGAMIHSRIGRVVFGVRNNKHGAAGSLMNVLNYPGMNHRVEITEGILADECAALLCDFYRMPRQVFNARKKAQSSINPGGSSGGSGGSETPGTSESATPENSGGSSGSSAKNTITKTLKLRIVRPYNSAEVEKIVADEKNNREKIALEKNKDKVKEACSKHLKVAAYCTTQVERNACLFCKARRLDDKFYQKLRGQFPDAVFWQEIGEIFRQLQKQAAEIYNQSLIELYYEIFIKGKGFANASSVEHYLSDVCYTRAAELFKNAAIASGLRGKVKSNFRLKELKNMKSGLPTTKSDNFPIPLVKQKGGQYTGFEISSHNDDFIIKIPFGRWQVKKEIDKYRPWEKFDFEQVRKSPKPISLLLSTQRRKRNKGWSKDEGTEAEIRKVMNGDYQTSYIEVKRGSKIGEKSAWMLNLSIDVPKIDKGVDPSIIGGIDVGVKSPLVCAINNVLSRYSISDNDLFHFNKKMFARRRILLKKNGHKRAGHGAKNKLKPISILTEKSKRFRKKLIERWACEIADFFIKNKVGTVQMENLESMKRREDSYFNIRLRGFWPYAEMQNKIEFKLKQYGIEIRKVAPNNTSKTCSKCGHLNNYFNFEYRKKNKFPHFKCEKCNFKENADYNAALNISNPELKSTKEEP

SEQ ID NO: 1398 - protein, 726 aa, synthetic construct
SEVEFSHEYWMRHALTLAKRARVEREVPVGAVLVLNNRVIGEGWNRAIGLHDPTAHAEIMALRQGGLVMQNYRLTDATLYVTFEPCVMCAGAMIHSRIGRVVFGVRNSKRGAAGSLMNVLNYPGMNHCVEITEGILVDECAALLCDFYRMPRQVLNAQKKAQSSISSGGSSGGSGGSEPPGASESVTPKSSAGSSAGSTKNTITKTLQLRIVRPYNSAEVEKIVTDEKNNREKIALEKNKDKVKEACSKHLKVAAYCTTQVERNACLFCKARRLDDKFYQKLRGQFPDAVFWQEIGEIFRQLQKQAAEIYNQSLIELYYEIFIKGKGITNASRVEHYLSDVCYTRAAELFKNAAIASGLRGKVKSNFRLKELKNMKSGLPTTKSDNFPIPLVKQKGGQYTGFEISSHNDDFIIKIPFGRWQVKEEIDKYRPWEKFDFEQVRKSPKPISLLLSTQRRKRNKGWSKDESTEAEIRKVMNGDYQTSYIEVKRGSKIGEKGAWMLSLSIDVPKIDKGVDPSIIGGIDVGVKSPLVCAINNALSRYSISDNDLFHFNKKMFARRRILLRKNRHKRAGHGARNKLKPITVLTEKSERFRKKLIERWACEIANFFIKNKVGTVQMENLESMKRREDSYFNIRLRGFWPYAEMQNKIEFKLKQYGIEIRKVAPNNTSKTCSKCGHLNNYFNFEFRKKNKFPHFKCEKCNFKENADYNAALNISNPKLKSTKEEP

SEQ ID NO: 1399 - protein, 726 aa, synthetic construct
SEVEFSHEYWMRHALTLAKRARDEREVPVGAVLVLNNRVIGEGWNRAIGLHDPTAHAEIMALRQGGLVMQNYRLIDATLYVTFEPCVMCAGAMIHSRIGRVVFGVRNNKHGAAGSLVNVLNYPGMNHRVEITEGILADECAALLCGFYRMPRQVFNARKKAQSSINPGGSSGGSSGSETPGTSESPTPESSGGSSGGSAKNTITKTLKLRIVRPYNSAEVERIVAEEKNNREKIALEKNKDKVKEACSKHLKVAAYCTTQVERNACLFCKARKLDDEFYQKLRGQFPDAVFWQEIGEIFRQLQKQAAEIYNQSLIELYYEIFIKGKGFANASSVEHYLSDVCYTRAAELFKNAAIASGLRGKVKSNFRLKELKNMKSGLPTTKSDNFPIPLVKQKGGQYTGFEISSHNDDFIIKIPFGRWQVKKEINKYRPWEKFDFEQVRKSPKPISLLLSTQRRKRNKGWSKDEGTEAEIRRVMNGDYQTSYIEVKRGSKIGEKSAWMLNLSIDVPKIDKGVDPSIIGGIDVGVKSPLVCAINNAFSRYSISDNDLFHFNKKMFARRRILLGKNRHKRAGHGVKNKLKPITILTEKSGRFRKKLIERWACEIADFFVKNKVGTVQMENLESMKRKEDSYFNIRLRGFWPYAEMQNKIEFKLKQYGIKVRRVAPNNTSKTCSKCGHLNNYFSFEYRKKNKFPHFKCEKCNFKENADYNAALNISNPKLKSTKEEP

SEQ ID NO: 1400 - protein, 726 aa, synthetic construct
SEVEFSHEYWMRHALTLAKRARDEREVPVGAVLVLNNRVIGEGWNRAIGLHDPTAHAEIMALRQGGLVMQNYRLIDATLYVTFEPCVMCAGAMIHSRIGRVVFGVRNSKHGAAGSLVNVLNHPGMNHRVEITEGILADECAALLCDFYRMPRQVFNARKKAQSSINPGGSSGGSSGSETPGTSESATPESSGGSSGGSAKNTITKTLKLRIVRPYNSAEVEKIVADEKNNREKTALEKNKDKVKEACSEHLKVATYCTTQVERNACLFCKARKLDDKFYQKLRGQFPDAVFWQEIGEIFRQLQKQAAEIYNQSLIELYYEIFIKGKGFANASSVEHYLSDVCYTRAAELFKNAAIASGLRNKTKSNFRLKELRSMKSGLPTTKSDNFPIPLVKQKGGQYTGFEISNHNSDFIIKIPFGRWQAKKEIDKYRPWEKFDFEQVRKSPKPISLLLSTQRRKRNKGWSKDEGTEAEIEKVMNGDYRTSYIEVKRGSKTGGKSAWMLNLSIDVPKIDKGVDPCIIGGIDVGVKSPLVCAINDAFSRYSISDNDLFHFNKKMFARRRILLKKNGHKRAGHGAKNKLKPITIMTEKGKRFRKKLIERWACEIADFFIKNKVGTVQMENLESMKRKEDSYFNIRLRGFWPYAEMQNKIEFKLKQYGIVVRKVAPNNTSKTCSKCGHLNNYFNFEYRKKNKFPYFKCEKCNFKENADYNAALNISNPQLKSTKGEP

SEQ ID NO: 1401 - protein, 726 aa, synthetic construct
SEVEFSHEYWMRHALTLAKRARDEREVPVGAVLVLNNRVIGEGWNRAIGLHDPTAHAEIMALRQGGLVMQNYRLTDATLYVTFEPCVMCAGAMIHSRIGRVVFGVRNSKRGAAGSLMNVLNYPGMNHCVEIMEGILVDECAALLCDFYRMPRQVLSAQKEAQSSISSGGSSGGSGGSETPGASGSVTPKSSVGSPAGSTKNTITKTLQLRIVRPYNSAEVEKIVADEKNNREKIALEKNKDKVKEACSKHLKVASYCTTRVERNACPFCKARKLDDKFYQKLRGQFPDAVFWQELGEIFRQLQRQAAEIYNQSLIELYYEIFIKGRGFANASSVEHYLSDVCYTRAAELFKNAAIASGLRGKVKGNFRLKELKNMKSGLPTTKSDNFPIPLVKQKGGQYTGFEISSHNDDFIIKIPFGRWQAKKEIDKYRPWEKFDFEQVRKSPKPISLLLSTQRRKRNKGWSKDEGTEAEIRRVMNGDYQTSYIEVKRGSKIGEKSAWMLNLSIDVPKIDKGVDPSIIGGIDVGVKSPLVCAINNAFSRYSISDNDLFHFNKKMFARRRILLKKNRHRRAGHGAKNKLKPISILTEKSKRFRKKLIERWACEIADFFIKNKVGTVQMENLESMKRKEDSYFNIRLRGFWPYAEMQNKIEFKLKQYGIEIRKVAPNNTSKTCSRCGHLNNYFNFEYRRKNKFPHFKCEKCNFKENADYNAALNISNPKLKSTKEEP

SEQ ID NO: 1402 - protein, 726 aa, synthetic construct
SEDEFSHEYWMRHALTLAKRARDEREVPVGAILVLNNRVIGEGWNRAIGLHDPTAHAEIMALRQGGLVMQNYRLIDATLYVTFEPCVMCAGAMIHSRIGRVVFGVRNSKHGAAGSLMNVLNYPGMNHRVEITEGILADECAALLCDFYRMPHQVLNARKKAQSSINPGGSSGGSSGSKTPGTSESATPESSGGSSGGSAKNSITKTLKLRIVRPYNSAEVEKIVADEKNNREKIALEKNKGKVKEACSKHLKVATYCTTQVERNACLFCKARKLDDKFYQKLRGQFPDAVFWQEIGEIFRQLQKQAAEIYNQSLIELYYEIFIKGKGFANASSVEHYLSDVCYTRAAELFKNAAIASGLRGKVKSNFRLKELKNMKSGLPTTKSDNFPIPLVKQKGGQYTGFEISSHNDDFIIKIPFGRWQVKKEIDRYRPWEKFDFEQVRKSPKPISLLLSTQRRKRNKGWSKDEGTEAEIRKVMNGDYQTSYIEVKRGSKIGEKSAWMLSLSIDVPKIDKGVDPSTIGGIDVGVKSPLVCAINNAFCRYSISDNDLFHFNKKMFARRRILLKKSRHKRAGHGAKNKLKPISILTEKSKRFRKKLIERWACEIADFFIKNKVGTVQMENLESMKRKEDSYFNIRLRGFWPYAEMQNKIEFKLKQYGIEIRKVAPNNTSKTCSKCGHLNNYFNFEYRKKNKFPHFKCEKCNFKENADYNAALNISNPKLKSTKEEP

SEQ ID NO: 1403 - protein, 726 aa, synthetic construct
SEVEFSHEYWMRHALTLAKRARDEREVPVGAILVLNNRIIGEGWNRAIGLHDPTAHAEIMALRQGGLVMQNYRLIDATLYVTFEPCVMCAGAMIHSRIGRVVFGVRNSKHGAAGSLVNVLNYPGMNHRVEITEGILVDECAALLCDFYRMPRQVFNARKKAQSSINPSGSSGGSSGSVTPGTSESATPESSGGGFGGSAKNTITKTLQLRIVRPYNSAEVEKIVADEKNNREKIALEKNKDKVKEACSKHLKVAAYCTTQVERNACLFCKARRLDDKFYQKLRGQFPDAVFWQEIGEIFRQLQKQAAEIYNQSLVELYYEILIKGKGIANASSVEHYLSDVCYTRAAELFKNAAIASGLRNKIKSNFRLKELRNMRSGLPTTKSDNFPIPLVKQKGGQYTGFEICSHNDDFIIKIPFGRWQVKKGIDKYRPWEKFDFEQVRKSPKPISLLLSTQRRKRNKGWSMDEGTEAEIRRVMNGDYQTSYIEVKRGSKIGEKSAWMLNLSIDVPKIDKGVDPCIIGGIDVGVKSPLVCAINNAFSRYSISDNDLFRFNKKVFARRRILLKKNRHRRAGHGAKNKLKPITILTEKSVRFRRKLIERWACEIADFFVKNKVGTVQMENLESMKRKEDSYFNIRLRGFWPYAEMQNKIEFKLKQYGIKIRKVAPNNTSKTCSKCGHLNNYFSFEYRKRNKFPHFKCEKCNFKEDADYNAALNISNPKLKSTKEGP

SEQ ID NO: 1404 - protein, 726 aa, synthetic construct; identical to SEQ ID NO: 684

SEQ ID NO: 1405 - protein, 726 aa, synthetic construct
SEVEFSHEYWMRHALTLAKRARDEREVPVGAVLVLNNRVIGEGWNRAIGQHDPTAHAEIMALRQGGLVMQNHRLVDATLYVTFEPCVLCAGAMVHSRIGRVVFGVRNSKRGAAGSLMNVLNYPGMNHRVEITEGILADECAALLCDFYRMPRQVFNARKKARSNINSGGSSGGSSGSETLGTREGATPESSGGSSGGSAKNTITKTLKLRIVRPYNSAEVEKIVADEKNNREKVALEKNKDKVKEACSKHLKVAAYCTTQVERNACLFCKARKLDDKFYQKLRGQFPDAVFWQEIGEIFRQLQKQAAEIYNQSLIELYYEIFIKGRGFANASSVEHYLSDVCYTRAAGLFKNAAIASGLRGKVKSNFRLKELKNMKSGLPTTKSDNFPIPLVKQKGGQYTGFEVSNRNDDFIIKIPFGRWQVKKEIDKYRPWEKFDFEQVRKSPKPISLLLSTQRRKRNKGWSKDEGTEAEIRKVMNGDYQTSYIEVKRGSKIGEKSAWMLNLSIDVPKIDKGVDPSIIGGIDVGVKSPLVCAINNSSSRYSICDNDLFRFNKKMFARRRILLKKNRHKRAGHGAKNKLKPITILTKKSERFRKKLIERWVCEVADFFIKNKVGTVQMENLESMKRKEDSYFNIRLRGFWPYAEMQNRIELKLKQYGIEIRRVAPNNTSRTCSKCGHLNNYFSFEYRKKSKFPHFKCEKCNFREDADYNAALNISNPKLKSTKEEP

SEQ ID NO: 1406 - protein, 726 aa, synthetic construct
SEVEFSHEYWMRHALTLAKRARDEREVPVGAVLVLNNRVIGEGWNRAIGLHDPTAHAEIMALRQGGLVMQNYRLTDATLYVTFEPCVMCAGAMIHSRIGRVVFGVRNSKRGAAGSLMNVLNYPGMNHCVEITEGILVDECAALLCDFYRMPRQVLNAQKRAQSSISSGGSSGGSSGSETPGASESVTPKGSGGSSAGSTKNTITKTLKLRIVRPYNSAEVEKIVADEKNNREKIALEKNKDKVKEACSKHLKVASYCTTQVERNACLFCKARKLDDKFYQKLRGQFPDAVFWQELGEIFRQLQKQAAEIYNQSLIELYYEIFIKGKGFANASSVEHYLSDVCYTRAAELFKNAAIASGLRGKVKSNFRMKELKNMKSGLPTTKSDNFPIPLVKQKGGQYTGFEISSHNDDFIIKIPFGRWQVKKEIDKYRPWEKFDFEQVRKSPKPLSLLLSTQRRKRNKGWSKDEGTEAEIRKVMNGDYQTSYIEVKRGSKIGEKSAWMLNLSIDVPKIDKGVDPSIIGGIDVGVKSPLVCAINNAFGRYSISDNDLFRYNKKMFARRRILQKKNRYKRAGHGAKNKLKPISILTEKSKRFRKKLIERWACEIADFFIKNKVGTVQMENLESMKRKEDSYFNIRLRGFWPYAEMQDKIEFKLKQYGIEIRKVAPNNTSKTCSRCGHLNNYFNFEYRRKNKFPHFKCEKCNFKENADYNAALNISNPKLKSTKEEP

SEQ ID NO: 1407 - protein, 726 aa, synthetic construct
SEVEFSHEYWMRHALTLARRARDEREVPVGAVLVLNNRVIGEGWNRAIGLHDPTAHAEIMALRQGGLVMRNYRLTDATLYVTFEPCVMCAGAMIHSRIGRVVFGVRNNKHGAAGSLVNVLNYPGMNHRVEITEGILADECAALLCDFYRMPRQVFNARKKTQSSINPGGSSGGSSGSETPGTSVSATPESSGSSSGGSAKNTITKTLKLRIVRPYNSAEVEKIVADEKNNREKIALEKNKDKVKEACSKHLKVASYCTTQVERNACPFCKARKLDDKFYQKLRGQFPDAVFWQELGEILRQLQKQAAEIYNQSLIELYYEIFIKGRGFANASSVEHYLSDVCYTRAAELFKNAAIASGLRGKVKSNFRLKELKNMKSGLPTTKSDNFPIPLVKQKGGQYTGFEISSHNDDFIIKIPFGRWQVRKEIDKYRPWEKFNFEQVRKSPKPISLLLSTQRRKRNKGWSKDEGTEAEIRRVMNGDYQTSYIEVKRGSKIGEKSAWMLNLSIDVPKIDKGVDPSIIGGIDVGVKSPLVCAINNAFSRYSISDNDLFHFNKKMFARRRILLKKNRRRRAGHGAKNKLKPITILTEKSVRFRKKLIERWACEIADFFIKNKVGTVQMENLESMKRKEDSYFNIRLRGFWPYAEMQNKIEFKLKQYGIEVRKVAPNNTSKTCSKCGHLNNYFNFEYRKKNKFPHFKCEKCNFKENADYNAALNISNPKLKSTKEEP

SEQ ID NO: 1408 - protein, 726 aa, synthetic construct
SEVEFSHEYWMRHALTLAKRARDEREVPVGAILVLNNRVIGEGWNRAIGLNDPTAHAEIMALRQGGLVMQNYRLIDATLYVTFEPCVMCAGAMIHSRIGRVVFGVRNNKHGAAGSLVNVLNYPGMNHRVEITEGVLADECAALLCDFYRMPRQVFNARKKAQSSINPGGSSGGSGGSETPGTSESATPESSGGSSGSSAKNTITKTLKLRIVRPYNSAEVEKIVADEKNNREKIALEKNKDKVKEACSKHLKVATYCTTQVERNACLFCKARRLDDKFYQKLRGQFPDAVFWQEIGEIFRQLQKQAAEIYNQSLVELYYEILIKGKGIANASSVEHYLSDVCYTRAAELFKNAAIASGLRNKIKSNFRLKELRNMKSGLPTTKSDNFPIPLVRQKGGQYTGFEISNHDGDFIIKIPFGRWQVKKEINKHRPWEKFDFEQVRKSPKPISLLLSTQRRKRNKGWSKDEGTEAEIRKVMNGDYRTSYIEVKRGSKIGEKSAWMLNLSIDVPKIDKGVDPSIIGGIDVGVKSPLVCAINNALSRYSISDNDLFHFNKKMFARRRILLRKNGHKRAGHGAKNKLKPITIMTEKSKRFRKKLIERWACEIADFFIKNKVGTVQMENLESMKRKEDSYFNIRLRGFWPYAEMQNKIEFKLKQYGIVVRKVAPNNTSKTCSQCGHLNNYFNFEYRKKNQFPYFKCEKCNFKENADYNAALNISNPQLKSTKGEP

SEQ ID NO: 1409 - protein, 726 aa, synthetic construct
SEVEFSHEYWMRHALTLAKRARDEREVPVGAVLVLNNRVIGEGWNRAIGLHDPTAHAEIMALRQGGLVMQNHRLIDATLYVTFEPCVLCAGAMVHSRIGRVVFGVRNSKRGAAGSLMNVLNYPGMNHRVEITEGVLADECAALLCDFYRMPRQVFNAQKKAQSSISPGGSSGGSSGSETPGASESVTPKSSGGSSGGSAKNTITKTLKLRIVRPYNSAEVEKIVADEKNNREKIALEKNKDKVKEACSKHLKVAAYCTTQVERNACLFCKARRLDDKFYQKLRGQFPDAVFWQEIGEIFRQLQKQAAEVYNQSLVELYYEILIKGKGIANASSVEHYLSDVCYTRAAELFKNAAIASGLRNKIKSNFRLKELRNMKSGLPTTKSDNFPIPLVRQKGGQYTGFEISNHDGDFIIKIPFGRWQVKKEINKHRPWEKFDFEQVRKSPKPISLLLSTQRRKRNKGWSKDEGTEAEIRKVMNGDHQTSYIEVKRGSKIGEKSAWMLNLSIDVPKIDKGVDPSIIGGIDVGVKSPLVCAIDNAFSRYSISDNDLFRFNKKMFARRRILLGKNRHKRAGHGVKNKLKPITILTEKSGRFRKKLIERWACEIADFFIKNKVGTVQMENLESMKRKEDSYFNIRLRGFWPYAEMQNKIEFKLKQYGIEIRKVAPNNTSKTCSKCGHLNNYFSFEFRKKNKFPHFKCEKCNFKEDADYNAALNISNPKLKSTKEEP

SEQ ID NO: 1410 - protein, 726 aa, synthetic construct
SEVEFSHEYWMRHALTLAKRARDEREVPVGAILVLNNRVIGEGWNRAIGLHDPTAHAEIMALRQGGQVMQNYRLIDATLYVTFEPCVMCAGAMIHSRIGRVVFGVRNSKHGAAGSLVNVLNYPGMNHRVEITEGILADECAALLCDFYRMPRQVFNARKKAQSSINPSGSSGGSSGSVTPGTSESATPESSGGSSAGSAKDTITKTLKLRIVRPYNSAEVEKIVADEKNSREKIALEKNKDKVKEACSKHLKVASYCTTQVERSACPFCKARKLDDKFYQKLGGQFPDAVFWQELGEILRQLQKQAAEIYNQSLIELYYEIFIKGRGFANASSVEHYLSDVCYTRAAELFKNAAIASGLRGKVKSNFRLKELKNMKSGLPTTKSDNFPIPLVKQKGGQYTGFEISSHNDDFIIKIPFGRWQVKKEIDKYRPWEKFDFEQVRKSPKPISLLLSTQRRKRNKGWSKDEGTEAEIRKVMNGDYQTSYIEVKRGSKTGEKSAWMLNLSIDVPKIDKGVDPSIIGGIDVGVKSPLVCAINNALSRYSISDNDLFRFNKKMFARRRILLKKNRHKRAGHGAKNKLKPISILTGKGERFRKKLIERWACEIADFFIKNKVGTVQMENLESMKRKEDSYFNIRLRGFWPYAEMQNKIEFKLKQYGIEIRKVAPNNTSKTCSKCGHLNSYFNFEYRKKNKFPHFKCEKCNFKENADYNAALNISNPKLKSTKEEP

SEQ ID NO: 1411 - protein, 726 aa, synthetic construct
SEVEFSHEYWMRHALTLAKRARDEREVPVGAVLVLNNRVIGEGWNRAIGLHDPTAHAEIMALRQGGLVMQNYRLIDATLYVTFEPCVMCAGAMVHSRIGRVVFGVRNSKRGAAGSLMNVLDYPGMGHRVEITEGILADECAALLCDFYCMPRQVFNAQKRAQSSINSGGSSGGSSGSETPGTSESATPESSGGGSSGSAKNTITKTLQLRIVRPYNSAEVEKIVADEKNNREKIALEKNKDKVKEACSRHLKVASYCTTQVERNACPFCKARKLDDKFYQKLRGQFPDAVFWQELGEILRQLQKQAAEIYNQSLIELYYEIFIKGRGFANAGSVEHYLSDVCYTRAAGLFKNAAIASGLRGKVKSNFRLKELKNMKSGLPTTKSDNFPIPLVKQKGGQYTGFEISSHNDDFIIKIPFGRWQVKKEIDKYRPWEKFDFEQVRKSPKPISLLLSTQRRKRNKGWSKDEGTEAEIRKVMNGDYQTSYIEVKRGSKIGEKSAWMLNLSIDVPKIDKGVDPSIIGGIDVGVKSPLVCAINNAFSRYSISDNDLFHFNKKMFARRRILLKKNRHKRAGHGAKNKLKPISILTGKSERFRKKLIERWACEIADFFIKNKVGTVQMENLESMKRKEDSYFNIRLRGFWPYAEMQNRIEFKLKQYGIEIRKVAPNNTSKTCSKCGHLNNYFNFEFRKKNKFPHFKCEKCNFKEDADYNAALNISNPKLKSTKEEP

SEQ ID NO: 1412 - protein, 726 aa, synthetic construct
SEVEFSHEYWMRHALTLAKRARDEREVPVGAILVLNNRVIGEGWNRAIGLHDPTAHAEIMALRQGGLVMQNYRLIDATLYVTFEPCVMCAGAMIHSRIGRVVFGVRNNKHGAAGSLVNVLNYPGMNHRVEITEGILADECATLLCDFYRMPRQVFNARKKAQSSINPGGSSGGSSGSETPGTGESATPESSGGSSGGSAKNTITKTLKLRIVRPYNSAEVEKIVADEKNNREKIALEKNKDKVKEACSKHLKVASYCTTQVERNACPFCKARKLDDKFYQKLRGQFPDAVFWQELGEILRQLQRQAAEIYNQSLIELYYEIFIKGRGFANASSVEHYLSDVCYTRAAELFRNAAIASGLRGKVKSNFRLKELKNMKSGLPTTKSDNFPIPLVKQKGGQYTGFEISSHNDDFIIKIPFGRWQVKKEIDKYRPWEKFDFEQVRKSPKPISLLLSTRRRKRNKGWSKDEGTEAEIRKVMNGDYQTSYIEVKRGSKIGEKSAWMLNLSIDVPKIDKGVDPSIIGGIDVGVKSPLVCAINNAFSRYSISDNDLFHFNKKMFARRRILLKKNRHKRAGHGAKNKLKPISILTEKSKRFRKKLIERWACEIADFFIKNKVGTVQMENLESMKRKEDSYFNIRLRGFWPYAEMQNKIEFKLKQYGIEIRKVAPNNTSKTCSKCGHLNNYFNFEYRRKNKFPHFKCEKCNFKEDADYNAALNISNPKLKSTKEEP

SEQ ID NO: 1413 - protein, 726 aa, synthetic construct
SEVEFSHEYWMRHALTLAKRARAEREVPVGAILVLNNRVVGEGWNRAIGLHDPTAHAEIMALRQGGLVMQNYRLTDATLYVTFEPCVMCAGAMIHSRIGRVVFGVRNNKHGAAGSLVNVLNYPGMNHRVEITEGILADECAALLCDFYRMPRQVFNARKKAQSSINPGGSSGGSSGSETPGTSESAAPESSGGSSGGSAKNTITKTLKLRIVRPYNSAEVEKIVADEKNNREKIALEKNKDKVKEACSKHLKVAAYCTTQVERNACLFCKARKLDDKFYQKLRGQFPDAVFWQELGEIFRQLQKQAAEIYNQSLIELYYEIFIKGKGFANASSVEHYLSDVCYTRAAELFKNAAIASGLRGKVKSNFRLKELKNMKSGLPTTKSDNFPIPLVKQKGGQYTGFEISSHNDDFTIKIPFGRWQVKKEIDKYRPWEKFDFEQVRKSPKPISLLLSTQRRKRNKGWSKDEGTEAEIRKVMNGDYQTSYIEVKRGSKIGEKSAWMLNLSIDVPKIDKGVDPSIIGGIDVGVKSPLVCAINNAFSRYSISDNDLFHYNKKMFARRRILLKKNRHKRAGHGAKNKLKPISILTEKSKRFRKKLIERWACEIADFFIKNKVGTVQIENLESMKRKEDSYFNIRLRGFWPYAEMQNKIEFKLKQYGIEIRKVAPNNTSKTCSKCGHLNSYFNFEYRKRNKFPHFRCEKCNFRENADYNAALNISNPKLRSTKEEP

SEQ ID NO: 1414 - protein, 726 aa, synthetic construct
SEVEFSHEYWMRHALTLAKRARDEREVPVGAVLVLNNRVIGEGWNRAIGLHDPTAHAEIMALRQGGLAMQNYRLVDATLYVTFEPCVLCAGAMVHSRIGRVVFGVRNSKRGAAGSLMNVLNHPGMNHRVEITGGILADECAALLCDFYRMPRQVFNAQKKARSNINSGGSSGGSSGSETPGTSESATPESSGGSSAGSTKNTITKTLKLRIVRPYNSAEVEKIVADEKNSREKIALERNKGKVKEACSEHLKVAAYCTTQVERNACLFCKARKLDDRFYQKLRGQFPDAVFWQETGEIFRQLQRQAAEIYNQSLIELYYEIFIKGKGFANASRVEHYLSDVCYTRAAELFKNAAIASGLRSKVRSNFRLKELKNMKSGLPTTKSDNFPIPLVKQKGGQYTGFEISSHNDDFVIKIPFGRWQVKEEIDKYRPWEKFDFEQVRKSPKPISLLLSTRRRKRNKGWSKDEGTEAEIRRVMNGDYQTSYIEVKRGSKIGEKSAWMLSLSIDVPKIDKGVDPRIIGGIDVGVKSPLVCAISNAFSRYSISDNDLFHFNKKMFARRRILLKKSKHKRAGHGAKNKLKPITIMTEKSERFRKKLIERWACEIANFFIKNKVGTVQMENLEGMKRKEDSYFNIRLRGFWPYAEMQNKIEFKLKQYGIVVRKVAPNNTSKTCSKCGHLNNYFNFEFRKKNKFPHFKCEKCNFKENADYNAALNISNPKLKSTKEEP

SEQ ID NO: 1415 - protein, 726 aa, synthetic construct
SEVEFSHEYWMRHALTLAKRARDEREVPVGAILVLNNRVIGEGWNRAIGLHDPTAHAEIMALRQGGLVMQNYRLIDATLYVTFEPCVMCAGAMIHSRIGRVVFGVRNNKHGAAGSLVNVLNYPGMNHRVEITEGILADECAALLCDFYRMPRQVFNARKKAQSSINPGGSSGGSSGSETPGTSESATPESSGGSSGGSAKNTITKTLKLRIVRPYNSAEVEKIVADEKDNREKIALEKNKDKVKEACSKHLKVAAYCTTQVERNACLFCKARKLDDKFYQKLRGQFPDAVFWQEIGEIFRQLQKQAAEIYNQSLIELYYEIFIKGKGFANASSVEHYLSDVCYTRAAELFKNAAIASGLRGKVKSNFRLKELKNMKSGLPTTKSDNFPIPLVKQKGGQYTGFEISSHNDDFIIKIPFGRWQVKKEINKYRPWEKFDFEQVRKSPKPISLLLSTQRRKRNRGWSKDEGTEAEIKKVMNGDYQTSYIEVKRGSKIGEKSAWMLNLSIDVPKIDKGVDPSIIGGIDVGVKSPLVCAINNAFSRYSISDNDLFHFNKKMFARRRILLKKGKHKRAGHGAKNKLKPITILTEKSGRFRKKLIERWACEIAGFFIKNKVGTVQMENLESMKRKEDSYFNIRLRGFWPYAEMQNKIEFKLKQYGIEIRKVAPNNTSKTCSKCGHLNNYFNFEYRKKNKFPHFKCEKCNFKEDADYNAALNISNPKLKSTKEEP

SEQ ID NO: 1416 - protein, 726 aa, synthetic construct
SEAEFSHEYWMRHALTLAKRARDEREVPVGAVLVLNDRVIGEGWNRAIGLHDPTAHAEIMALRQGGLVMQNYRLTDATLYVTFEPCVMCAGAMIHSRIGRVVFGVRNSKRGAAGSLMNVLNYPGMNHCVEITEGILVDECAALLCDFYRMPRQVLNAQKKAQSSISSGGSSGGSSGSETPGTSESPTPESSGGSPGGSAKNTLTKTLKLRIVRPYNSAEVEKIVADEKNNRERIALEKNKDKVKEACSKHLKVAAYCTTQVERNACLFCKARKLDDKFYQKLRGQFPDAVFWQETGEIFRQLQRQAAEIYNQSLIELYYEIFIKGKGFANASSVEHYLSDVCYTRAAELFKNAAIASGLRGKVKSNFRLKELKNMKSGLPTTKSDNFPIPLVKQKGGQYTGFEISSHNDDFIIKIPFGRWQAKKEIDKYRPWEKFDFEQVRKSPKPISLLLSTRRRKRNKGWSKDEGTEAEIRRVMNGDYQTSYIEVKRGSKIGEKSAWMLNLSIDVPKIDKGVDPSIIGGIDVGVKSPLVCAINNAFSRYSISDNDLFHFNKKMFARRRILLKKNRHKRAGHGAKNKLKPISILTERSKRFRKKLIERWACEIADFFIKNKVGTVQMENLESMKRKEDSYFNIRLRGFWPYAEMQNKIEFKLKQYGIEIRKVAPNNTSKTCSKCGHLNNYFNFEYRRKNKFPHFKCEKCNFKENADYNAALNISNPKLKSTKEEP

SEQ ID NO: 1417 - protein, 726 aa, synthetic construct
SEVEFSHEYWMRHALTLAKRARDEREVPVGAVLVLNNRVIGEGWNRAIGLHDPTAHAEIMALHQGGLVMQNYRLIDATLYVTFEPCVMCAGAMIHSRIGRVVFGARNSKRGAAGSLMNVLSYPGMNHRVEITEGILADECAALLCDFYRMPRQVFNAQKKAQSSINSGGSSGGGSGSETPSTSESTTPKNSGGSSAGSAKNTITKTLKLRIVRPYNSAEVEKIVADEKNNREKIALEKNKGKVKEACRKHLKVAAYCTTQVERNACLFCRARKLDDKFYQKLRGQFPDAVFWQEIGEIFRQLQKQAAEIYNQSLIELYYEIFIKGKGFANASSVEHYLSDVCYTRAAELFKNAAIASGLRGKVKSNFRLKELKNMKSGLPTTKSDNFPIPLVKQKGGQYTGFEISNHNSDFIIKIPFGRWQAKKEIDRYRPWEKFDFEQVRKSPKPISLLLSTQRRKKNGGWSKDEGTEAEIKKVMNGDYQTSYIEVKRGSKIGEKSAWMLSLSIDVPKIDKGVDPSIIGGIDVGVKSPLVCAISNAFSRYSISDNDLFHFNKKMFARRRILLKKSRHKRAGHGAKNKLKPITILTEKSRRFRKKLIERWACEIADFFIKNKVGTVQMENLESMKRREDSYFNIRLRGFWPYAEMQNKIEFKLKQYGIEVRKVAPNNTSKTCSKCGHLNNYFNFEYRKKNKFPHFKCGKCNFEENADYNAALNISNPKLKRAKEEP

SEQ ID NO: 1418 - protein, 726 aa, synthetic construct
SEVEFSHEYWMRHALTLAKRARDEREVPVGAILVLNNRVIGEGWNRAIGLHDPTAHAEIMALRQGGLVMQNYRLIDATLYVTFEPCVMCAGAMIHSRVGRVVFGVRNSKHGAAGSLMNVLNYPGMNHRVEITEGILADECAALLCDFYRMPRRVFNARKKAQSSIDPGGPSGSSSSSETPGTSESATPESSGGSSGGSAKNTITKTLKLRIVRPYNSTEVEKIVADEKNNREKIALEKNKDKVKEACSKHLKVASYCTTQVERNACLFCKARKLDDKFYQKLRGQFPDAVFWQELGEIFRQLQKQAAEIYNQSLIELYYEIFIKGKGFANASSVEHYLSDVCYTRAAELFKNAAIASGLRGKVKSNFRLKELKNMKSGLPTTKSDNFPIPLVKQKGGQYTGFEISNHNSDFIIKIPFGRWQVKKEINKYRPWEKFDFEQVRKSPKPISLLLSTQRRKRNKGWSKDEGTEAEIRRVMNGDYQTSYIEVKRGSKIGEKSAWMLSLSIDVPKIDRGVDPSIIGGIDVGVKSPLVCAINNAFGRYSISDNDLFHFNKKMFARRRILLKKNRHKRAGHGAKNKLKPITILTEKSGRFRKKLIERWACEIADFFIKNKVGTVQMENLEGMKRKEDSYFNIRLRGFWPYAEMQNKIEFKLKQYGIEIRKVAPNNTSKTCSKCGHLNNYFNFEYRKKNKFPHFKCEKCNFKENADYNAALNISNPKLKSTKEEP

SEQ ID NO: 1419 - protein, 726 aa, synthetic construct
SEVEFSHEYWMRHALTLAKRARDEREVPVGAVLVLNNRVIGEGWNRAIGLHDPTAHAEIMALRQGGLVMQSYRLTDATLYVTFEPCVMCAGAMIHSRIGRVVFGVRNSKRGAAGSLMNVLNYPGMNHCVEITEGILVDECAALLCDFYRMPRQVLNAQKKAQSSISPGGSSGGSSGSETPGASGSVTPKSSGGSSAGSTKNTITKTLQLRIVRPYNSAEVEKIVADEKNNREKIALEKNKDKVKEACSKHLKVAAYCTTQVERNACLFCKARKLDDKFYQKLRGQFPDAVFWQEIGEIFRQLQKQAAEIYNQSLIELYYEIFIKGKGFANASSVEHYLSDVCYTRAAELFKNAAIASGLRGKVKSNFRLKELKNMRSGLPTTKSDNFPIPLVRQKGGQYTGFEISNHDGDFIIKIPFGRWQVKKEINKHRPWEKFDFEQVRKSPKPISLLLSTQRRKRNKGWSKDEGTEAEIRKVMNGDYQTSYIEVKRGSKIGEKSAWMLNLSIDVPKIDKGVDPGIIGGIDVGVKSPLVCAINNASSRYSISDNDLFHFNKKMFARRRILLKKNRHKRAGHGAKNKLKPITIMTEKSKRFRKKLIERWACEIADFFIKNKVGTVQMENLESMKRKEDSYFNIRLRGFWPYAEMQNKIEFKLKQYGIEIRKVAPNNTSKTCSKCGHLNNYFNFEYRKKNKSPHFKCEKCNFKEDADYNAALNISNPKLKSTKEEP

SEQ ID NO: 1420 - protein, 726 aa, synthetic construct
SEVEFSHEYWMRHALTLAKRARDEREVPVGAVLVLNNRVIGEGWNRAIGLHDPTAHAEIMALRQGGLVMQNYRLVDATLYVTFEPCVLCAGAMVHSRIGRVVFGVRNSKRGAAGSLMNVLNYPGMNHRVEITEGILADECAALLCDFYRMPRQVFNARKKAQSSINPGGSSGGSGGSETPGASGSPTPESSGGSSGGSAKNTITKTLKLRIVRPYNSAEVERIVADEKNNREKIALEKNKDKVKEACSKHLKVAAYCTTRVERNACLFCKARRLDDKFYQKLRGQFPDAVFWQEIGGIFRQLQKQAAEVYNQSLVELYYEILIKGKGIANASSVEHYLSDVCYTRAAELFKNAAIASGLRNKIKSNFRLKELRNMKSGLPTTKSDNFPIPLVRQKGGQYTGFEISNYNGDFIIKIPFGRWQVKKEINKHRPWEKFDFEQVRKSPKPISLLLSTQRRKRNKGWSRDEGTEAEIRKVMNGDYQTSYIEVKRGSKIGEKSAWMLNLSIDVPKIDKGVDPSIIGGIDVGVKSPLVCAINNAFSRYSISDNDLFRFNKKVFARRRILLKKNRHKRAGHGTKNKLKPITILTEKSGRFRKKLIERWACEIANFFIKNKVGTVQMENLESMKRKGDSYFNIRLRGFWPYAEMQNRIELKLKQYGIEIRKVAPNNTSKTCSKCGHLNNYFNFEYRKKNKFPHFKCEKCNFKEDADYNAALNISNPKLKSTREEP

SEQ ID NO: 1421 - protein, 726 aa, synthetic construct
SEVEFSHEYWMRHALTLAKRARDEREVPVGAILVLNNRVIGEGWNRAIGLHDPTAHAEIMALRQGGLVMQNYRLIDATLYVTFEPCVMCAGAMIHSRIGRVVFGVRNNKHGAAGSLVNVLDYPGMNHRVEITEGILADECAALLCDFYCMPRQVFNAQKRAQSSINSGGSSGGSSGSETPGTSESATPESSGGGSSGSAKNTITKTLQLRIVRPYNSAEVEKIVADEKNNREKIALEKNKDKVREACSKHLKVASYCTTQVERNACPFCKARKLDDKFYQKLRGQFPDAVFWQELGEILRQLQKQAAEIYNQSLIELYYEIFIKGRGFANASSVEHYLSDVCYTRAAELFKNAAIASGLRGKVKSNFRLKELKNMKSGLPTTKSDNFPIPLVKQKGGQYTGFEISSHNDDFIIKIPFGRWQAKKEIDKYRPWEKFDFEQVRKSPKPISLLLSTQRRKRNRGWSKDEGTEAEIRKVMNGDYQTSYIEVKRGSKTGEKSAWMLNLSIDVPKIDKGVDPSIIGGIDVGVKSPLVCAINNAFSRYSISDNDLFRFNKKMFARRRILLKKNRHKRAGHGAKNKLKPITILTEKSRRFRKKLIERWACEIADFFIKNKVGTVQMESLESMKRKEDSYFNIRLRGFWPYAEMQNKIEFKLKQYGIEIRKVAPNNTSKTCSKCGHLNNYFNFEYRKKNKFPHFKCEKCYFKENADYNAALNISNPKLKSTKEEP

SEQ ID NO: 1422 - protein, 726 aa, synthetic construct
SEVEFSHEYWMRHALTLAKRARDEREVPVGAVLVLNNRVIGEGWNRAIGLHDPTAHAEIMALRQGGLVMQNHRLADATLYVTFEPCVLCAGAMVHSRIGRVVFGVRNSKRGAAGSLMNVLNYPGMNHRVEITEGILADECAALLCDFYRMPRQVFNAQKKAQSSISSGGSSGGSSGSETPGAGESVTPKSSVGSSAGSTKNTITKTLKLRIVRPYNSAEVEKIVADEKNNREKIALEKNKDKVKEACSKHLKVAAYCTTQVERNACLFCKARKLDDKFYQKLRGQFPDAVFWQEVGEIFRQLQKQAAEIYNRSLIELYYEIFIKGKGFANASSVEHYLSDVCYTRAAELFKNAAIASGLRGKVKSNFRLKELKNMKSGLPTTKSDNFPIPLVKQKGGQYTGFEISSHNDDFIIKIPFGRWQVRKEIDKYRPWEKFNFEQVRKSPKPISLLLSTRRRKGNKGWSKDEGTEAEIRKVMNGDYRTSYIEVKRGSKTGEKSAWMLNLSIDVPKIDKGVDPSIIGGIDVGVKSPLVCAINNAFSRYSISDNDLFHFNKKMFARRRILLKKNRHKRAGHGAKNKLKPITIMTEKSKRFRKKLIERWACEIADFFIKNKVGTVQMENLESMKRKEDSYFNIRLRGFWPYAEMQNKIEFKLKQYGIVVRKVAPNNTSKTCSKCGHLNNYFNFEYRKKNKFPHFKCERCNFKENADYNAALNISNPRLKSTKEEP

SEQ ID NO: 1423 - protein, 726 aa, synthetic construct
SEVEFSHEYWMRHALTLAKRARDEREVPVGAVLVLNNRAIGEGWNRAIGLHDPTAHAEIMALRQGGLVMQNYRLTDATLYVTFEPCVMCAGAMIHSRIGRVVFGVRNSKRGAAGSLMNVLNYPGMNHRVEITEGILADECAALLCDFYRMPRHVLNAQKRAQSSISSGGSSGGCSGSEMPGASESVTPKSSGGSSGGSAKNTITKTLKLRIVRPYNSAEVEKIVADEKNNREKIALEKNKDKVKEACNKHLKVAAYCTTQVERNACLFCKARKLDDKFYQKLRGQFPDAVFWQEIGEIFRQLQKQAAEIYNQSLIELYYEIFIKGKGFANASSVEHYLSDVCYTRAAELFKNAAIASGLRGKVKSNFRLKELKNMKSGLPTTKSDNFPIPLVKQKGGQYTGFEISNLNSDFIIKIPFGRWQVKKEINKYRPWEKFDFEQVRKSPKPISLLLSTQRRKRNKGWSKDEGTEAEIRKVMNGDYQTSYIEVKRGSKIGEKSAWMLNLSIDVPKIDKGVDPSIIGGIDVGVKSPLVCAINNAFSRYSISDNDLFHFNKKMFARRRILLKKNRHKRAGHGAKNKLRPITILAEKSERFRKKLIEKWACEIADFFIKNKVGTVQMENLESMKRKEDSYFNIRLRGFWPYAEMQNKIEFKLKQYGIEIRKVAPNNTSKTCSKCGHLNNYFNFEYRKKNKFPHFKCEKCNFKENADYNAALNISNPKLKSTKEEP

SEQ ID NO: 1424 - protein, 726 aa, synthetic construct
SEVEFSHEYWMRRALTLAKRARDEREVPVGAVLVLNNRVIGEGWNRAIGLHDPTAHAEIMALRQGGLVMQNHRLTDATLYVTFEPCVMCAGAMIHSRIGRVVFGVRNSKRGAAGSLMNVLNYPGMNHCVEITEGILVDECAALLCDFYRMPRQVLSAQKKAQSSINSGGSSGGSCGSETPGTSESATPESSGGSSGGSAKNTITKTLQLRIVRPYNSAEVEKIVADEKNNREKAALEKNKDKVKEACSKHLKVAAYCTTQVERNACLFCKARKLDDKFYQKLRGQFPDAVFWQEVGEIFRQLQKQAAEIYNQSLIELYYEIFIKGKGFANASSVEHYLSDVCYTRAAELFKNAAIASGLRGKVKSNFRLKELKNMKSGLPTTKSDNFPIPLVKQKGGQYTGFEISNRNSDFIIKIPFGRWQVKKEINKYRPWEKFDFEQVRKSPKPISLLLSTQRRKRNKGWSKDEGTEAEIRKVMNGDYQTSYIEVKRGSKTGEKSAWMLNLSIDVPKIDKGVDPSIIGGIDVGVKSPLVCAINNAFSRYSISDNDLFRFNKKMFARRRILLMKNRHKRAGHGAKNKLKPISILTGKSERFRKKLIERWACEIADFFIKNKVGTVQMENLESMKRKEDSYFNIRLRGFWPYAEMQNKIEFKLKQYGIEIRKVAPNNTSKTCSKCGHLNNYFNFEYRKKNKFPHFKCEKCNFKENADYNAALNISNPKLKSTKEEP

SEQ ID NO: 1425 - protein, 726 aa, synthetic construct
SEVEFSHEYWMRHALTLAKRARDECEVPVGAILVLNNRVIGEGWNRAIGLHDPTAHAEIMALRQGGLVMQNYRLIDATLYVTFEPCVMCAGAMVHSRIGRVVFGVRNSKRGAAGSLMNVLNYPGMNHRVEITEGILADECAALLCDFYRMPRQVFNARKRARSNINSGGSSGGSSGSETLGTREGATLESSGGSSGGSAKNTITKTLKLRIVRPYNSAEVEKIVADEKNNREKIALEKNKDKVKEACSKHLKVAAYCTTQVERNACLFCKARKLDDKFYQKLRGQFPDAVFWQEIGEIFRQLQRQAAEIYNQSLIELYYEILIKGKGFANASSVEHYLSDVCYTRAAELFKNAAIASGLRGKVKSNFRLKELKNMKSGLPTTKSDNFPVPLVKQKGGQYTGFEISSHNDDFIIKIPFGRWQVKKEIDKYRPWEKFDFEQVRKSPKPISLLLSTQRRKRNKGWSKDEGTEAEIRKVMNGDYQTSYVEVKRGSKTGEKSAWMLSLSIDVPKIDKGVDPSIIGGIDVGVKSPLVCAINNAFSRYSISDNDLFRFNKKMFARRRILLKKNRHKRAGHGAKNKLKPITILTEKSRRFRKKLIERWACEIADFFIKNKVGTVQMENLESMKRREDSYFNIRLRGFWPYAEMQNKIEFKLKQYGIEIRKVAPNNTSKTCSKCGHLNNYFNFEYRKKNQFPHFKCEKCNFKEDADYNAALNISNPKLKSTKEEP

SEQ ID NO: 1426 - protein, 726 aa, synthetic construct
SEVEFSHEYWMRRALTLAKRARDEREVPVGAVLVLNNRVIGEGWNRAIGLHDPTAHAEIMALRQGGLVMQNYRLTDATLYVTFEPCVMCAGAMIHSRIGRVVFGVRNSKRGAAGSLMNVLNYPGMNHCVEITEGILVDECAALLCDFYRMPRQVLSAQKKAQSNISSGGSSGGSSGSETPGARGSVTPKSSVGSSAGSTKNTITKTLKLRIVRPYNSAEVEKIVADEKNNREKIALEKNKDKVKEACSKHLKVASYCTTQVERNACPFCKARKLDDKFYQKLRGQFPDAVFWQELGEIFRQLQKQAAEIYNQSLIELYYEIFIKGKGITNASRVEHYLSDVCYTRAAELFKNAAIASGLRSKVRSNFRLKELKNMKSGLPTTKSDNFPIPLVKQKGGQYTGFEISSHNDDFIIKIPFGRWQVKKEIDKYRPWEKFDFEQVRKSPKPISLLLSTQRRKRNKGWSKDEGTEAEIRKVMNGDYQTSYIEVKRGSKTGEKSAWMLNLSIDVPKIDKGVDPSIIGGIDVGVKSPLVCAINNAFSRYSISDNDLFRFNKKMFARRRILLKKNRHKRAGHGAKNKLKPISILTGKSERFRKKLIERWACEIADFFIKNKVGTVQMENLESMKRKEDSYFNIRLRGFWPYAEMQNKIEFKLKQYGIEIRKVAPNNTSKTCSKCGHLNNYFNFEYRKKSKFPHFKCEKCNFKENADYNAALNISNPKLKSTKEEP

SEQ ID NO: 1427 - protein, 726 aa, synthetic construct
SEVEFSHEYWMRHALTLAKRARDEREVPVGAILVLNNRVIGEGWNRAIGLHDPTAHAEIMAMRQGGLVLQNYRLIDATLYVTFEPCVMCAGAMIHSRIGRVVFGVRNNKHGAAGSLVNVLNYPGMNHRVEITEGILADECAALLCDFYRMPRQVFNARKKAQSSINPGGSSGGSSGSETPGTSESATPESSGGSSGSSAKNTITKTLKLRIVRPYNSAEVEKIVADEKNNREKIALEKNKDKVKEACSKHLKVASYCTTQVERNACLFCKARKLDDKFYQKLRGQFPDAVFWQELGEILRQLQKQAAEIYNQSLIELYYEIFIKGRGFANASSVEHYLSDVCYTRAAELFKNAAIASGLRGKVKSNFRLKELKNMKSGLPTTKSDNFPIPLVKQKGGQYTGFEISSHNDDFIIKIPFGRWQVKKEIDKYRPWEKFDFEQVRKSPKPISLLLSTQRRKRNKGWSKDEGTEAEIRKVMNGDYQTSYIEVKRGSKTGEKSAWMLNLSIDVPKIDKGVDPSIIGGIDVGVKSPLVCAINNAFSRYSISDNDLFRFNKKMFARRRILLKKNRHKRAGHGAKNKLKPISILTEKSERFRKKLIERWACEIADFFIRNKVGTVQMENLEGMKRKEDSYFNIRLRGFWPYAEMQNKIEFKLKQYGIEVRKVAPNNTSKTCSKCGHLNNYFNFEYRKKNKFPHFRCEKCNFKENADYNAALNISNPKLKSTKEEP

SEQ ID NO: 1428 - protein, 726 aa, synthetic construct
SEVEFSHEYWMRHALTLAKRARDEREVPVGAVLVLNNRVIGEGWNRTTGLHDPTAHAEIMALRQGGLVMRNYRLTDATLYVTFEPCAMCAGAMIHSRIGRVVFGVRNSKRGAAGSLMNVLNYPGMNHCVEITEGILVDECAALLCDFYRMPRQVLNAQKKAQSSISPGGSSGGSSGGKAPGTSESATLESSGGSSGGSAKNSITKTLKLRIVRPYNSAEVEKIVADEKNNREKIALEKNKGKVKEACSKHLKVATYCTTQVERNACLFCRARKLDDKFYQKLRGQFPDAVFWQEIGEIFRQLQKQAAEIYNQSLIELYYEIFIKGKGITNASRVEHYLSDVCYTRAAELFKNAAIASGLRSKVRSNFRLKELKNMKSGLPTTKSDNFPIPLVKQKGGQYTGFEISSHNSDFIIKIPFGRWQVKEEIDKYRPWEKFDFEQVRKSPKPISLLLSTQRRKKNKGWSKDEGTEAEIRRVMNGDYQTSYIEVKRGSKIGEKSAWMLNLSIDVPKIDKGVDPSIIGGIDVGVKSPLVCAINNALSRYSISDNDLFHFNKKMFARRRILLRKNRHKRAGHGAKNKLKPITIMTEKSKRFRKKLIERWACEIADFFIKNKVGTVLMENLESMKRREDSYFNIRLRGFWPYAEMQNKIEFKLKQYGIEVRKVAPNNTSKTCSRCGHLNNYFNFEYRKKNKFPLFKCEKCNFKENADYNAALNISNPKLKSTKEEP

SEQ ID NO: 1429 - protein, 726 aa, synthetic construct
SEVEFSHEYWMRHALTLAKRARDEREVPVGAVLVLNNRVIGEGWNRAIGLQDPTAHAEIMALRQGGLVMQNYRLSDATLYVTFEPCVMCAGAMIHSRIGRVVFGVRNSKRGAAGSLMNVLNYPGMNHCVEITEGILVDECAALLCDFYRMPRLVLSAQKKAQSSVSSGGSSGGSSGSETPGAGGSVTPKSSVGSSAGSTKNTITKTLKLRIVRPYNSAEVEKIVADEKNNREKIALEKNKGKVKEACSKHLKVATYCTTQVERNACLFCKARKLDDKFYQKLRGQFPDAVFWQEVGEIFRQLQKQAAEIYNQSLIELYYEIFIKGKGIANASSVGHYLSDVCYTRAAELFKNAAIASGLRGKIKSNFRLKELKNMKSGLPTTKSDNFPIPLVKQKGGQYTGFEISNHNGDFIIKIPFGRWQVKKEINKYRPWEKFDFEQVRKSPKPISLLLSTQRRKRNKGWSKDEGTEAEIKKVMNGDYQISYIEVKRGSKIGEKSAWTLNLSVDVPKIDKGVDPSIIGGIDVGVKSPLVCAINNALSRYSISDNDLFHFNKKVFARRRILLKKNRHRRAGHGAKNKLKPISILTEKSERFRKKLIERWACEIADFFIKNKVGTVQMENLESMKRREDSYFNIRLRGFWPYAKMQNKIEFKLKQYGIEIRKVAPNNTSKTCSKCGHLNNYFNFEYRKKNKFPHFKCEKCNFKENADYNAALNISNPKLKSTKEEH

SEQ ID NO: 1430 - protein, 726 aa, synthetic construct
SEVEFSHEYWMRHALTLAKRARDEREVPVGAILVLNNRVIGEGWNRAIGLHDPTAHAEIMALRQGGLVTQNYRLIDATLYVTFEPCVMCAGAMIHSRIGRVVFGVRNSKHGAAGSLVNVLNYPGMNHRVEITEGVLADECAALLCDFYRMPRQVFNARKKAQSNINPGGSSGGSSGSETPGTSDSATPGSSGGSSGGSAKNTITKTLKLRIVRPYNSAEVEKIVADEKNNREKTALEKNKDKVKEACSEHLKVATYCTTQVERNACLFCKARKLDDKFYQKLRGQFPDAVFWQEIGEIFRQLQKQAAEIYNQSLIELYYEIFIKGKGFANASSVEHYLSDVCYARAAELFKNAAIASGLRNKTKSNFRLKELRSMKSGLPTTKSDNFPIPLVKQKGGQYTGFEISNHNSDFIIKIPFGRWQAKKEIDKYRPWEKFDFEQVRKSPKPISLLLSTQRRKRNKGWSKDEGTEAEIEKVMNGDYQTSYIEVKRGSKTGGKSAWMLNLSIDVPKIDKGVDPSIIGGIDVGVKSPLVCAINDAFSRYSISDNDLFHFNKKMFARRRILLKKNGHKRAGHGAKNKLRPITIMTEKSKRFRKKLIERWACEIADFFIKNKVGTVQMENLESMKRKEDSYFNIRLRGFWPYAEMQNKIEFKLKQYGIVVRKVAPNNTSKTCSKCGHLNNYFNFEYRKKNKFPHFKCEKCNFKENADYNAALNISNPQLKSTKGEP

SEQ ID NO: 1431 - protein, 726 aa, synthetic construct
SEVEFSHEYWMRHALTLAKRARDEREVPVGAVLVLNNRVIGEGWNRAIGLHDPTAHAEIMALRQGGLVMQNYRLIDATLYVTFEPCVLCAGAMVHSRIGRVVFGVRNSKRGAAGSLMNVLNHPGMNHRVEITGGILADECAALLCDFYRMPRQVFNAQKKARSNINSGGSSGGSSGSETLGTSESATPESSGGSSGGSAKNTITKTLKLRIVRPYNSAEVEKIVADEKNNREKIALEKNKDKVKEACSKHLKVAAYCTTQVERNACLFCKARKLDDKFYQKLRGQFPDAVFWQEIGEIFRQLQKQAAEIYNQSLIELYYEIFIKGKGITNASRVEHYLSDVCYTRAAELFKNAAIASGLRSKVRSNFRLKELKNMKSGLPTTKSDNFPIPLVKQKGGQYTGFEISSHNDDFIIKIPFGRWQVKKEIDKYRPWEKFDFEQVRKSPKPISLLLSTQRRKRNKGWSKDEGTEAEIRKVMDGDYQTSYIEVKRGSKIGEKSAWMLNLSIDVPKIDKGVDPRIIGGIDVGVKSPLVCAINNVLSRYSISDNDLFHFNKKMFARRRILLKKNGHKRAGHGAKNKLKPITIMTEKSKRFRKKLIERWACEIADFFIKNKVGTVQMENLESMKRKEDSYFNIRLRGFWPYAEMQNKIEFKLKQYGIVVRKVAPNNTSKTCSQCGHLNNYFNFEYRKKNKFPHFKCEKCNFKEDADYNAALNISNPKLKSTKEEP

SEQ ID NO: 1432 - protein, 726 aa, synthetic construct
SEVEFSHEYWMRHALTLAKRARDEREVPVGAILVLNNRVIGEGWNRAIGLHDPTAHAEIMALRQGGLVLQDYRLIDATLYVTFEPCVMCAGAMIHSRIGRVVFGVRNNKHGAAGSLVNVLNYPGMNHRVEITEGILADECAALLCDFYRMPRQVFNARKKAQSSINPGGSSGGSSGSETPGTSESATPESSGGSSGSSAKNTITKTLKLRIVRPYNSAEVEKIVADEKNNREKIALEKNKDKVKEACSKHLKVAAYCTTQVERNACLFCKARRLDDKFYQKLRGQFPDAVFWQEIGEIFRQLQKQAAEIYNQSLVELYYEILIKGKGFANASSVEHYLSDVCYTRAAELFKNAAIASGLRGKVKSNFRLKELKNMKSGLPTTKSDNFPIPLVKQKGGQYTGFEISNHNSDFIIKIPFGRWQVKKEINKYRPWEKFDFEQVRKSPKPISLLLSTQRRKRNKGWCKDEGTEAEIRKVMNGDYQTSYIEVKRGSRIGEKSAWMLSLSIDVPKIDRGVDPSIIGGIDVGVKSPLVCAINNAFSRYSISDNDLFHFNKKMFARRRILLKKNRHKRAGHGAKNKLKPISVLTEKSKRFRKKLIERWACEIADFFIKNKVGTVQMENLESMKRKEDSYFNIRLRGFWPYAEMQNKIEFKLKQYGIKVRKVAPNNTSKTCSKCGHLNNYFSFEYRKKNKFPHFKCEKCNFKENADYNAALNISNPKLKSTKEEP

SEQ ID NO: 1433 - protein, 726 aa, synthetic construct
SEVEFSHEYWMRHALTLAKRARDEREVPVGAILVLNNRVIGEGWNRAIGLHDPTAHAEIMALRQGGLVMQNYRLIDATLYVTFEPCVMCAGAMIHSRIGRVVFGVRNSKHGAAGSLVNVLNYPGMNHRVEITEGVLADECAALLCDFYRMPRQVFNARKKAQSNINPDGSSGGSSGSETPGTSESATPGSSGGSSGGSAKNTITKTLKLRIVRPYNSAEVEKIVADEKNNRVKTALEKNKDKVKEACSEHLKVAAYCTTQVERNACLFCKARKLDDKFYQKLRGQFPDAVFWQEIGEIFRQLQKQAAEIYNQSLIELYYEIFIKGKGFANASSVEHYLSDVCYTRAADLFKNAAIASGLRGKVKSNFRLKELRNTKSGLPTTKSDNFPIPLVKQKGGQYTGFEISSHNDDFIIKIPFGRWQVKKEIDKYRPWEKFDFEQVRKSPKPISLLLSTQRRKRNKGWSKDEGTEAEIRKVMNGDYQTSYIEVKRGSKIGEKSAWMLNLSIDVPKIDKGVDPSIIGGIDVGVKSPLVCAINNAFSRYSISDNDLFHFNKKMFARRRILLKKNRHKRAGHGAKNKLKPISILTEKSKRFRKKLIERWACEIADFFIKNKVGTVQMENLESMKRKEDGYFNIRLRGFWPYAEMQNKIEFKLKQYGIEIRKVAPNNTSKTCSKCGHLNNYFNFEYRKMNKFPHFKCEKCNFKEDADYNAALNISNPKLKSTKEEP

SEQ ID NO: 1434 - protein, 726 aa, synthetic construct
SGVEFSHEYWMRHALTLAKRARDEREVPVGAVLVLNNRVIGEGWNRAIGLHDPTAHAEIMALRQGGLVLQNYRLIDATLYVTFEPCVMCAGAMIHSRIGRVVFGVRNSKHGAAGSLVNVLNYPGMNHRVEITEGILADECAALLCDFYRMPRQVFNARKKAQSSINPSGSSGGSSGSETPGTSESPTPESSGGSPGGSAKNTITKTLKLRIVRPYNSAEVEKIVADEKNNREKIALEKNKDKVKEACSKHLKVAAYCTTQVERNACLFCKARKLDDKFYQKLRGQFPDAVFWQEIGEIFRQLQKQAAEIYNQSLIELYYEIFIKGKGFANACSVEHYLSDVCYTRAAELFKNAAIASGLRGKVKSNFRLKELKNMKSGLPTTKSDNFPIPLVKQKGGQYTGFEISSHNSDFIIKIPFGRWQEKEEIDKYRPWEKFDFEQVRRSPKPISLLLSTQRRKKNKGWSKDEGTEAEIRKVMNGDYQTSYIEVKRGSKIGEKSAWMLNLSIDVPKIDKGVDPSIIGGIDVGVKSPLVCAINNAFSRYSISDNDLFRFNKKMFARRRILLGKNRHKRAGHGVKNKLKPITILTEKSGRFRKKLIERWACEIADFFVKNKVGTVQMENLESMKRKEDSYFNIRLRGFWPYAEMQNKIEFKLKQYGIKVRKVAPNNTSKTCSKCGHLNNYFSFEYRKKNKFPHFKCEKCNFKENADYNAALNISNPKLKSTKEEP

SEQ ID NO: 1435 - protein, 726 aa, synthetic construct
SEVEFSHEYWMRHALTLAKRARDEREVPVGAVLVLNNRVIGEGWNRAIGLHDPTAHAEIMALRQGGLVMQNYRLVDATLYVTFEPCVLCAGAMVHSRIGRVVFGVRNSKRGAAGSLMNVLNYPGMNHRVEITEGILADECAALLCDFYRMPRQVFNAQKKARSNINSGGSSGGSSGSETPGASESVTPKSSGGSSGGSTKNTITKTLKLRIVRPYNSAEVEKIVADEKNSREKIALERNKDKVKEACSKHLKVAAYCTTQVERNACLFCKARRLDDKFYQKLRGQFPDAVFWQEIGEIFRQLQKQAAEIYNQSLIELYYEIFIKGKGIAGASRVGHYLSDVCYTRAAELFKNAAIASGLRSKIKSNFRLKELKNMKSGLPTTKSDNFPIPLVKQKGGQYTGFEISSHNDDFIIKIPFGRWQVKKEIDKYRPWEKFDFAQVRKSPKPISLLLSTQRRKKNKGWSKDEGTEAEIRRVMNGDYQTSYVEVKRGSKTGEKSAWMLNLSIDVPKIDKGVDPSIIGGIDVGVKSPLVCAINNAFSRYSISDNDLFRFNKKMFARRRILLKKNRHKRAGHGAKNKLKPISILTEKSKRFRKKLIERWACEIADFFIKNKVGTVQMENLESMKRKEDSYFNIRLRGFWPYAEMQNKIEFKLKQYGIGIRKVAPNNTSRTCSKCGHLNNYFNFEYRRKNKFPHFKCEKCNFKENADYNAALNISNPKLKSTKEGP

SEQ ID NO: 1436 - protein, 726 aa, synthetic construct
SEVEFSHEYWMRHALTLAKRARDEREVPVGAILVLNNRVIGEGWNRAIGLHDPTAHAEIMALRQGGLVMQNYRLIDATLYVTFEPCVMCAGAMIHSRIGRVVFGVRNSKHGAAGSLVNVLNYPGMNHRVEITEGILADECAALLCNFYRMPRQVFNVRKKTQSSINPGGSSGGSSGSETPGTSESATPESSGSSSVGSAKNTITKTLKLRIVRPYNSAEVEKIVADEKNNREKIALEKNKDKVKEACSKHLKVAAYCTTQVERSACLFCKARRLDDKFYQKLRGQFPDAVFWQEIGEIFRQLQKQAAEIYNQSLIELYYEIFIKGKGFANASSVEHYLSDVCYTRAAELFKNAAIASGLRGKVKSNFRLKELKNMKSGLPTTKSDNFPIPLVKQKGGQYTGFEISSHNDDFIIKIPFGRWQVKKEIDKYRPWEKFDFEQVRKSPKPISLLLSTQRRKRNKGWSKDEGTEAEIRKVMNGDYQTSYIEVKRGSKIGEKSAWMLNLSIDVPKIDKGVDPSIIGGIDVGVKSPLVCAINNAFSRYSISDNDLFRFNKKVFARRRILLKKNRHKRAGHGTKNKLKPITILTEKSGRFRKKLIERWACEIADFFIKNKVGTVQMENLESMKRKEDSYFNIRLRGFWPYAEMQNKIEFKLKQYGIEIRRVAPNNTSRTCSKCGHLNNYFNFEYRRKYKFPHFKCEKCNFKEDADYNAALNISNPKLKSTKEEP

SEQ ID NO: 1437 - protein, 726 aa, synthetic construct
SEVEFSHEYWMRRALTLAKRARDEREVPVGAILVLNNRVIGEGWNRAIGLHDPTAHAEIMALRQGGLVMQNYRLIDATLYVTFEPCVMCAGAMIHGRIGRVVFGVRNSKHGAAGSLMNVLNYPGMNHRVEITEGILADECAALLCDFYRMPHRVLNARKKAQSSINPGGSSCGSSGSETPGTSESATPESSGGGSGGSTKNTITKTLKLRIVRPYNSAEVEKVVADEKNNREKTALEKNKDKVKEACSEHLKVASYCTTQVEGNACLFCKARKLDDKFYQKLRGQFPDAVFWQELGGIFRQLQKQAAEIYNQSLIELYYEIFIKGKGITNASRVEHYLSDVCYTRAAELFKNAAIASGLRSKVRSNFRLKELKNMKSGLPTTKSDNFPIPLVKQKGGQYTGFEISSHNSDFIIKIPFGRWQVKEEIDKYRPWEKFDFEQVRKSPKPISLLLSTQRRKKNKGWSKDEGTEAEIRRVMNGDYQTSYIEVKRGSKIGEKSAWMLNLSIDVPKIDKGVDPSIIGGIDVGVKSPLVCAINNSSSRYSICDNDLFRFNKKMFARRRILLKKNRHKRAGHGAKNKLKPITILTKKSERFRKKLIERWVCEVADFFIKNKVGTVQMENLESMKRREDSYFNIRLRGFWPYAEMQSKIEFKLKQYGIKIRKVAPNNTSKTCSKCGHLNNYFNFEFRKKNKFPHFKCEKCNFKEDADYNAALNISNPKLKGTKEEP

SEQ ID NO: 1438 - protein, 726 aa, synthetic construct
SEVEFSHEYWMRHALTLAKRARDEREVPVGAILVLNNRVIGEGWNRAIGLHDPTAHAEIMALRQGGLVMQNHRLVDATLYVTFEPCVMCAGAMIHSRIGRVVFGVRNSKRGAAGSLTNVLNYPGMNHRVEITEGILVDECAALLCDFYRMPRQVFNAQRKAQSTINSGGSSGGSSGSETPGTSESPTPESSGGSPGGSAKNTITKTLKLRIVRPYNSAEVEKIVADEKNNREKIALEKNKDKVKEACSKHLKVAAYCTTQVERNACLFCKARKLDDKFYQKLRGQFPDAVFWQEIGEIFRQLQKQAAEIYNQSLIELYYEIFIKGKGFANASSVEHYLSDVCYTRAAELFKNAAVASGLRGKVKSNFRLKELKNMKSGLPTTKSDNFPIPLVKQKGGQYTGFEISSHNDDFIIKIPFGRWQVKKEIDKYRPWEKFDFEQVRKSPRPISLLLSTQRRKRNKGWSKDEGTEAEIRRVMNGDYQTSYIEVKRGSKIGEKSAWMLNLSIDVPKIDKGVDPSIIGGIDVGVKSPLVCAINNAFSRYSISDNDLFHFNKKMFARRRILLKKNRHRRAGHGAKNKLKPITILTEKSKRFRKKLIERWACEIADFFVKNKVGTVQMENLESMKRKEDSYFNIRLRGFWPYAEMQNKIEFKLKQYGIEIRKVAPNNTSKTCSKCGHLNNYFNFEYRKRNKFPHFKCEKCNFKENADYNAALNICNPKLKSTKEEP

SEQ ID NO: 1439 - protein, 726 aa, synthetic construct
SEVEFSHEYWMRHALTLAKRARDEREVPVGAVLVLNNRVIGEGWNRAIGLHDPTAHAEIMALRQGGLAMQNYRLVDATLYVTFEPCIMCAGAMIHSRIGRVVFGVRNSKRGAAGSLMNVLNYPGTNHRVKITEGILADECAALICDYYRMPRQVFNARKKAQSSINSGGSSDGGSGSETPGTSESATPESSGGSSGGSAKNTITKTLKLRIVRPYNSAEVEKIVADEKNNREKIALEKNKDKVKEACSEHLKVAAYCTTQVERNACPFCKARKLDDKFYQRLRGQFPDAVFWQELGEILRQLQKQAAEIYNQSLIELYYEIFIKGRGFANASSVEHYLSDVCYTRAAELFKNAAIASGLRGKVKSNFRLKELKNMKSGLPTTKSDNFPIPLVKQKGGQYTGFEISSHNDDFIIKIPFGRWQVKKEIDKYRPWEKFDFEQVRKSPKPISLLLSTQRRQKNKGWSKDEGTEAEIRRVMNGDYQTSYIEVKGGGKIGEKSTWMLNLSIDVPKIDKGVDPSIVGGIDVGVKSPLVCAINNSFSRYSICDNDLFRFNKKMFARRRILLKKNRHKRAGHGAKNKLKPISILTGKSERFRKKLIERWACEIADFFIKNKVGTVQMENLESMKRKEDSYFNIRLRGFWPYAEMQNKIEFKLRQYGIEVRKVAPNNTSKTCSKCGHLNNYFNFEYRKKNKFPHFKCEKCNFKENADYNAALNISNPKLKSTKEVP

SEQ ID NO: 1440 - protein, 726 aa, synthetic construct
SEVEFSHEYWMRHALTLAKRARDEREVPVGAVLVLNNRVIGEGWNRAIGLHDPTAHAEIMALRQGGLVMQNYRLIDATLYVTFEPCVMCAGAMVHSRIGRVVFGVRNSKRGAAGSLMNVLDYPGMGHRVEITEGILADECAALLCDFYCMPRQVFNAQKRAQSSINSGGSSGGSSGSETPGTSESATPESSGGGSSGSAKNTITKTLQLRIVRPYNSAEVEKIVADEKNNREKIALEKNKDKVKEACSKHLKVAAYCTTQVERNACLFCKARRLDDKFYQKLRGQFPDAVFWQEIGEIFRQLQKQAAEVYNQSLVELYYEILIKGKGIANASSVEHYLSDVCYTRAAELFKNAAIASGLRNRIKSNFRLKELKNMKSGLPTTKSDNFPIPLVKQKGGQYTGFEISNHNSDFIIKIPFGRWQAKKEIDKYRPWEKFDFEQVRKSPKPISLLLSTQRRKRNRGWSKDEGTEAEVKKVMNGDYQISYIEVKRGSKIGEKSAWMLNLSIDVPKIDRGVDPSIIGGIDVGVKSPLVCAISNAFSRYSISDNDLFHFNKKMFARRRILLKKSKHRRAGHGAKNKLKPITILTEKSRRFRKKLIERWACEIADFFIKNKVGTVQMENLEGMKRKEDSYFNIRLRGFWPYAEMQNKIEFKLKQYGIEVRKVAPNNTSKTCSKCGHLNNYFNFEYRKKNKFPHFKCEKCSFKENADYNAALNISNPKLKSTKERP

SEQ ID NO: 1441 - protein, 726 aa, synthetic construct
SEDEFSHEYWMRHALTLAKRARDGREVPVGAVLVLNNRVIGEGWNRAIGLHDPTAHAEIMALRQGGLVMQNYRLIDATLYVTFEPCVMCAGAMVHSRIGRVVFGVRNSKRGAAGSLMNVLDYPGMGHRVEITEGILADECAALLCDFYCMPCQVFNAQKRAQSSINSGGSSGGSSGSDTPGTSESATPESSGGGSSGSAKNTITKTLQLRIVRPYNSAEVEKIVADEKNNREKIALEKNKDKVREACSKHLEVAAYCTTQVERNACLFCKARKLDDKFYQKLRGQFPDAVFWQELGEIFRQLQKQAAEIYNQSLIELYYEIFIKGKGFANASSVEHYLSDVCYTRAAELFKNAAIASGLRGKVKSNFRLKELKNMKSGLPTTKSDNFPIPLVKQKGGQYTGFEISSHNDDFIIKIPFGRWQAKKEIDRYRPWEKFDFEQVRKSPKPISLLLSTQRRKRNKGWSKDVGTEAEIRKVMNGDYQTSYIEVKRGSKIGEKSAWMLNLSIDVPKIDKGVDPSIIGGIDVGVKSPLVCAINNAFSRYSISDNDLFRFNKKMFARRRILLKKNRHQRAGHGAKNKLKPITILTEKSGRFRKKLIERWACEIADFFIKNKVGTVQMENLESMKRKEDSYFNIRLRGFWPYAEMQNKIEFKLKQYGIKIRKVAPNNTSKTCSKCGHLNNYFSFEYRKKNKFPHFKCEKCNFKENADYNAALNISNPKLMSTKEEP

SEQ ID NO: 1442 - protein, 726 aa, synthetic construct
SEVEFSHEYWMRHALTLAKRARDEREVPVGAILVLNNRVIGEGWNRAIGLHDPTAHAEIMALRQGGLVMQNYRLIDATLYVTFEPCVMCAGAMIHSRIGRVVFGVRNNKHGAAGSLVNVLNYPGMNHRVEITEGILADECAALLCDFYCMPRQVFNAQKRAQSSINSGGSSGGSSGSETPGTSESATPGSSGGSSGGSAKNTITKTLKLRIVRPYNSAEVEKIVADEKNNREKIALEKNKDKVKEACSKHLKVAAYCTTQVERNACLFCKARRLDDKFYQKLRGQFPDAVFWQEIGEIFRQLQKQAAEIYNQSLVELYYEILIKGKGIANASSVEHYLSDVCYTRAAKLFKNAAIASGLRNKIKSNFRLKELKNMKSGLPTTKSDNFPIPLVKQKGGQYTGFEISNHNGDFIIKIPFGRWQAKKEIDKYRPWEKFDFEQVRKSPKPISLLLSTQRRKRNRGWSRDEGTEAEVKKVMNGDYQISYIEVKRGSKIGEKSAWTLNLSIDVPKIDKGVDPSIIGGIDVGVKSPLVCAISNALSRYSINDNDLFHFNKKMFARRRILLKKSKHKRAGHGAKNKLKPITILTEKSRRFRKKLIERWACEIADFFIKNKVGTVQMENLEGMKRKEDSYFNIRLRGFWPYAEMQNKIEFKLKQYGIKIRKVAPNNTSKTCSKCGHLNNYFSFEYRKKNKFPHFKCEKCNFKEDADYNAALNISNPKLKSTKEEP

SEQ ID NO: 1443 - protein, 726 aa, synthetic construct
SEAEFSHEYWMRRALTLAKRARDEGEVPVGAVLVLNNRVIGEGWNRAIGLHDPTAHAEIMALRQGGLVMQNYRLVDATLYVTFEPCVLCAGAMVHSRIGRVVFGVRNSKRGAAGSLMNVLNYPGMNHRVEITEGILADECAALLCDFYRMPRQVFNAQKKARSNINSGSSSGGSSGSETPGTSESATPVSSSGSSGGSAKNTITKTLKLRIVRPYNSAEVEKIVADEKNNREKIALEKNKGKVEEACSKHLKVATYCTTQVERNACLFCKARKLDDKFYQKLRGQFPDAVFWQEIGEIFRQLQKQAAEIYNQSLIELYYEIFIEGKGSANARSVEHYLSDVCYTRAAELFKNAAIASGLRGKVKGNFRLKELKSMKSGLPTTKSDNFPIPLVKQKGGQYTGFEISSHNDDFIIKIPFGRWQVKKEIDKYRPWEKFDFEQVRKSPKPISLLLSTQRRKRNKGWSKDEGTEAEIRKVMNGDYQTSYIEVKRGSKIGEKSAWMLSLSIDVPKIDKGVDPSIIGGIDVGVKSPLVCAINNALSRYSISDNDLFHFNKKMFARRRILLRKNGHKRAGHGAKNKLKPITILTEKSVRFRKKLIERWACEIADFFIKNKVGTVQMENLESMKRKEDGYFNIRLRGFWPYAEMQNKIEFKLKQYGIEIRKVAPNNTSKTCSKCGHLNNYFNFEYRKKNKFPHFKCEKCNFREDADYNAALNISNPKLKSTKEEP

SEQ ID NO: 1444 - protein, 726 aa, synthetic construct
SEVEFSHEYWMRHALTLAKRARDEREVPVGAVLVLNNRVIGVGWNRAIGLHDPTAHAEIMALRQGGLVMQNYRLTDATLYVTFEPCVMCAGAMVHSRIGRVVFGVRNNKHGAAGSLVNVLNYPGMNHRVEITEGILADECAALLCDFYRMPRQVFNARKKAQSSINPGGSSGGSSGSGTPGTSESATPESSGGGSSGSAKNTITKTLQLRIVRPYNSAEVEKIVADEKNNREKIALEKNKDKVKEACSKHLKVASYCTTQVERNACPFCKARKLDDRFYQKLRGQFPDAVFWQETGEIFRQLQRQAAEIYNQSLIELYYEIFIKGRGFANASSVEHYLSDVCYTRAAELFKNAAIASGLRGKVKGNFRLKELKNMKSGLPTTKSDNFPIPLVKQKGGQYTGFEISSHNDDFIIKIPFGRWQVKKEIDKYRPWEKFDFEQVRKSPKPISLLLSTQRRKRNKGWSKDEGTEAEIRKVMNGDYQTSYIEVKRGSKIGEKSAWMLNLSIDVPKIDKGVDPSIIGGIDVGVKSPLACAINNAFSRYSISDNDLFRFNKKMFARRRILLGKNRHKRAGHGVKNKLKPITILTEKSGRFRKKLIERWACEIADFFVKNKVGTVQMENLESMKRKEDSYFNIRLRGFWPYAEMQNKIEFKLKQYGIKVRKVAPNNTSKTCSKCGHLNNHFSFEYRKKNKFPHFKCEKCNFKEDADYNAALNISNPKLKSTKEEP

SEQ ID NO: 1445 - protein, 725 aa, synthetic construct
SEDEFSHEYWMRHALTLAKRARDGREVPVGAVLVLNNRVIGEGWNRAIGLHDPTAHAEIMALRQGGLVMQNYRLTDATLYVTFEPCVMCAGAMIHSRIGRVVFGVRNNKRGAAGSLMNVLNYPGMNHCVEITEGILVDECAALLCDFYRMPCQVLNAQKKAQSSISSGGSSGGSSGSDTLGASEGVTPKSSVGSSASSTKNTITKTLKLRIVRPYNSAEVEKIVADEKDNREKIALEKNRDKVKEACSKHLKVAAYCTTQVERNACLFCKARKLDDKFYQKLRGQFPDAVFWQEIGEIFRQLQKQAAEIYNQSLIELYYEIFIKGKGFANASSVEHYLSDVCYTRAAELFKNAAIASGLRGKVKSNFRLKELKNMKSGLPTTKSDNFPIPLVKQKGGQYTGFEVSSHNDDFIIKIPFGRWQVKKEIDKYRPWEKFDFEQVRKNPKPISLLLSTQRRKRNKGWSKDEGTEAEIRKVMNGDYQTSYIEVKRGNKVGEKSAWMLNLSIDAPKIDKGVDPSIIGGIDVGVKSPLVCAINNAFSRYSISDNDLFRFNKKVFARRRILLKKNRHKRAGHGTKNKLKPITILTEKSGRFRKKLIERWACEIANFFIKNKVGTVQMENLESMKRKEDSYFNIRLRGFWPYAEMQNKIEFKLKQYGIEIRKVAPNNTSKTCSKCGHLNNYFSFEYRKKNKFPHFKCEKCNFKEDADYNAALNISNPKLSTKEVL

SEQ ID NO: 1446 - protein, 726 aa, synthetic construct
SEVEFSHEYWMRHALTLAKRARDEREVPVGAILVLNNRVIGEGWNRAIGLHDPTAHAEIMALRQGGLVMQNYRLIDATLYVTFEPCVMCAGAMVHSRIGRVVFGVRNSKRGAAGSLMNVLDYPGMGHRVEITEGILADECAALLCDFYRMPRQVFNAQKRAQSSINSGGSSGGSSGSETLGASESATPESSGGGSSGSAKNTITKTLQLRIVRPYNSAEVEKIVADEKNNREKIALEKNKDKVREACSKHLKVAPYCTTQVERNACPFCKARKLDDKFYQKLRGQFPDAVFWQELGEILRQLQKQAAEIYNQSLIELYYEIFIKGKGFANASSVEHYLSDVCYTRAAELFKNAAIASGLRGKVKSNFRLKELKNMKSGLPTTKSDNFPIPLVKQKGGQYTGFEISSHNDDFIIKIPFGRWQVKKEIDKYRPWEKFDFEQVRKSPKPISLLLSTQRRKRNRGWSKDEGTEAEIRKVMNGDYQTSYIEVKRGSKIGEKSAWMLNLSIDVPEIDKGVDPSIIGGIDVGVRSPLVCAINNAFSRYSIGDNDLFRFNKKMFARRRILLKKNRHKRAGHGAKNKLKPITILTEKSRRFRKKLIERWACEIADFFIKNKVGTVQMESLESMKRKEDSYFNIRLRGFWPYAEMQNRIEFKLKQYGIEIRRVAPNNTSRTCSKCGHLNNYFNFEYRKKNKFPHFKCEKCNLREDADYNAALNISNPKLKSIKEEP

SEQ ID NO: 1447 - protein, 726 aa, synthetic construct
SEVEFSHEYWMRHALTLAKRARDGREVPVGAVLVLNNRVIGEGWNRAIGLHDPTAHAEIMALRQGGLVMQNYRLIDATLYVTFEPCVMCAGAMIHSRIGRVVFGVRNNKHGAAGSLVNVLDYPGMNHRVEITEGILADECAALLCDFYRMPRQVFNARKKAQSSISPGGSSGGSSGSETPGTSESATPESSGGSPGGSAKNTITKTLKLRIVRPYNSAEVEKIVADEKNNREKIALEKNKDKVKEACSKHLKVAAYCTTQVERNACLFCKARKLDDKFYQKLRGQFPDAVFWQEIGEVFRQLQKQAAEIYNQSLIELYYKIFIKGKGFANASSVEHYLSDVCYTRAAELFKNAAIASGLRGKVKSNFRLKELKNMKSGLPTTKSDNFPIPLVKQKGGQYTGFEIGSHNDDFIIKIPFGRWLAKKEIDKYRPWEKFDFEQVRKSPKPISLLLSTQRRKRNRGWSKDEGTEAEIRKVMNGDYQTSYIEVKRGSKIGEKSAWMLNLSIDVPKIDKGVDPSIIGGIDVGVKSPLVCAINNAFSRYSISDNDLFRFNKKMFARRRILLGKNRHKRAGHGVKNKLKPITVLTEKSKRFRKKLIERWACEIADFFIKNKVGTVQMENLESMKRKEDSYFNIRLRGFWPYAEMQNKIEFKLKQYGIEIRKVAPNNTSKTCSKCGHLNNYFNFEYRKKNKFPHFKCEKCNFKENADYNAALNISNPKLKSTKEEP

SEQ ID NO: 1448 - protein, 726 aa, synthetic construct
SEVESSHEYWMRHALALAKRARDEREVPVGAVLVLNNRVIGEGWNRAIGLHDPTAHAEIMALRQGGLVMQNYRLTDATLYVTFEPCVMCAGAMIHSRIGRVVFGVRNNKHGAAGSLVNVLNYPGMNHRVEITEGILADECAALLCDFYRMPRQVFNARKKARSNINSGGSSGRSSGGETPGASGSVTPKSSGGSSAGSAKDTITKTLKLRIVRPYNSAEVEKIVADEKNSREKIALEKNKDKVKEACSEHLKVAAYCTTQVERNACLFCKARKLDDGFYQKLRGQFPDAVFWQEIGEIFRQLQKQAAEIYNQSLIELYYEIFIKGKGFANASSVEHYLSDVCYTRAAELFKNAAIASGLRNKIKSNFRLKELKNMKSGLPTTKSDNFPIPLVRQKGGKYTGFEISSHNDDFIIKIPFGRWQVKKEIDKYRPWEKFDFEQVRRSPKPISLLLSTQRRKKNKGWSKDEGTEAEIRRVMNGDYQTSYVEVKRGSKIGEKSAWMLNLSIDVPKIDKGVDPSIIGGIDVGVKSPLVCAINNAFSRYSISDNDLFHFNKKMFARRRILLKKNRRRRAGHGAKNKLKPITILTEKSVRFRKKLIERWACEIADFFIKNKVGTVQMENLESMKRKEDSYFNIRLRGFWPYAEMQNKIEFKLKQYGIKIRKVAPNNTSRTCSKCGHLNNYFSFEYRKKNKFPHFKCEKCNFKEDADYNAALNISNPKLKGTKEEP

SEQ ID NO: 1449 - protein, 726 aa, synthetic construct; identical to SEQ ID NO: 807

SEQ ID NO: 1450 - protein, 726 aa, synthetic construct
SEDEFSHEYWMRHALTLAKRARDGREVPVGAVLVLNNRVIGEGWNRAIGLHDPTAHAEIMALRQGGLVMQNYRLIDATLYVTFEPCVMCAGAMVHSRIGRVVFGVRNSKRGAAGSLMNVLDYPGMGHRVEITEGILADECAALLCDFYCMPRQVFNAQKRAQSSINSGGSSGGSSGSETPGTSESAIPGSSGGGSSGSAKNTITKTLQLRIVRPYNSAEVEKIVADEKNNREKIALEKNKDKVKEACSKHLKVASYCTTQVERNACPFCKARKLDDKFYQKLRGQFPDAVFWQELGEILRQLQKQAAEIYNQSLIELYYEIFIRGRGFANASSVEHYLSDVCYTRAAELFKNAAIASGLRGKVKSNFRLKELKNMKSGLPTTKSDNFPIPLVKQKGGQYTGFEISNHNDDFIIKIPFGRWQVKKEIDKYRPWEKYDFEQVRKSPKPISLLLSTQRRKRSKGWSKDEGTEAEIRKVMNGDYQTSYIEVKRGSKTGEKSAWMLNLSIDVPKIDKGVDPSIIGGIDVGVKSPLVCAINNAYSRYSISDNDLFRFNKKMFARRRILLRKNRHKRAGHGAKNKLKPISILTGKSERFRKKLIERWACEIADFFIKNRVGTVQMENLESMKRKEDSYFNIRLRGFWPYAEMQNKIEFKLKQYGIEIRKVAPNNTSKTCSKCGHLNNYFNFEYRKKNKFPHFKCEKCNFKENADYNAALNISNPKLKSTKEEP

SEQ ID NO: 1451 - protein, 726 aa, synthetic construct
SEDEFSHEYWMRHALTLAKRARDGREVPVGAVLVLNNRVIGEGWNRAIGLHDPTAHAEIMALRQGGLVMQNYRLIDATLYVTFEPCVMCAGAMVHSRIGRVVFGVRNSKRGAAGSLMNVLDYPGMNHRVEITGGILADECAALLCDFYRMPRRVFNAQKKAQPSINSGGSSGGSSGSVTPGTSEGATPESSGGSSGGSAKNTITKTLKLRIVRPYNSAEVEKIVADEKNNREKIALEKNKDKVKEACSKHLKVAAYCTTQVERNACQFCKARKLDDKFYQKLRGQFPDAVFWQEIGEIFRQLQKQAAEIYNQSLIELYYEIFIKGKGFANASSVEHYLSDVCYTRAAELFKNAAIASGLRGKVKSNFRLKELKNMKSGLPTTKSDNFPIPLVKQKGGQYTGFEISNHNGDFIIKIPFGRWQVKKETDKYRPWEKFDFEQVRKSPKPISLLLSTQRRKRNKGWGKDEGTEAEIRRVMNGDYQTSYIEVKRGSKIGEKSAWMLNLSIDVPKIDKGVDPSIIGGIDVGVKSPLVCAINNAFSRYSISDNDLFHFNKKMFARRRILLKRNRHKRAGHGAKNKLKPITTLTEKSKRFRKKLIERWACEIADFFIKNKVGTVQMENLESMKRKEDSYFNIRLRGFWPYAEMQNKIEFKLRQYGIEIRKVAPNNTSKTCSKCGHLNNYFNFEYRKKNKFPHFKCEKCDFEENADYNAALNISNPKLKNTKGEP

SEQ ID NO: 1452 - protein, 726 aa, synthetic construct
SEVEFSHEYWMRHALTLAKRARDEREVPVGAILVLNNRVIGEGWNRAIGLHDPTAHAEIMALRQGGLVMQNYRLIDATLYVTFEPCVMCAGAMIHSRIGRVVFGVRNSKHGAAGSLVNVLNYPGMNHRVEITEGILADECAALLCDFYRMPRQVFSARRKAQSSISPGGSSGGSSGGETPGSSKSLTPESPGGSSGGSAKNTITKTLKLRIVRPYNSAEVEKIVADEKNNREKIALEKNKDKVKEACGKHLKVAAYCTTQVERNACLFCKARKLDDKFYQKLRGQFPDAVFWQEIGEIFRQLQKQAAEIYNRSLIELYYEIFIKGKGFANASSVEHYLSDVCYTRAAELFKNAAIASGLRGKVKSNFRLKELKSMKSGLPTTKSDNFPIPLVKQKGGQYTGFEISSHNDDFIIKIPFGRWQVKKEIDKYRPWEKFDFEQVRKNPKPISLLLSTQRRKRNKGWSKDEGTEAEIRKVMNGDYQTSYIEVKRGSKIGEKSAWMLNLSIDVPKIDKGVDPSIIGGIDVGVKSPLVCAINNAFSRYSISDNDLFRFNKKVFARRRILLKKNRHKRAGHGTKNKLKPITILTEKSGRFRKKLIERWACEIANFFIKNKVGTVQMENLEGMKRKEDSYFNIRLRGFWPYAEMQNKIEFKLKQYGIKIRKVAPNNTSKTCSKCGHLNNYFNFEYRKKNKFPHFKCEKCNFKENADYNAALNISNPKLKSTKEEP

SEQ ID NO: 1453 - protein, 726 aa, synthetic construct
SEVEFSHEYWMRHALTLAKRARDEREVPVGAVLVLNNRVIGEGWNRAIGLHDPTAHAEIMALRQGGLVMQNYRLIDATLYVTFEPCVMCAGAMIHSRIGRVVFGVRNSKHGAAGSLVNVLNYPGMNHRVEITEGILADECAALLCDFYRMPRQVFNARKKAQPSINPGGSSGGSSGSVTPGTSESATPVSSSGSFGGSAKNTITKTLRLRIVRPYNSAEVEKIVADEKNNREKIALEKNKDKVKEACSKHLKVAAYCTTQVERNACLFCKARKLDDKFYQKLRGQFPDAVFWQEIGEIFRQLQKQAAEIYNQSLIELYYEIFIKGKGFANASSVEHYLSDVCYSRAAELFKNAAVASGLRGKVKSNFRLKELKNMKSGLPTTKSDNFPIPLVKQKGGQYTGFEISSHNDDFIIKIPFGRWQVKKEIDKYRPWEKFDFEQVRKSPKPISLLLSTQRRKRNKGWSKDEGTEAEIRKVMNGDYQTSYIEVKRGSKTGEKSAWMLNLSIDVPKIDKGVDPCIIGGIDVGVKSPLVCAINNAFSRYSISDNDLFHFNKKMFARRRILLKENGHKRAGHGAKNKLKPITIMTEKSKRFRKKLIERWACEIADFFIKNKVGTVQMENLESMKRKEDSYFNIRLRGFWPYAEMQNKIEFKLKQYGIVVRKVAPNNTSKTCSECGHLNNYFNFEYRKKNKFPHFKCEKCNFKENADYNAALNISNPKLKSTKEGP

SEQ ID NO: 1454 - protein, 726 aa, synthetic construct
SEVEFSHEYWMRHALTLAKRARDEREVPVGAVLVLNNRVIGEGWNRAIGLHDPTAHAEIMALRQGGLVLQNYRLVDATLYVTFEPCVLCAGAMVHSRIGRVVFGARNSKRGAAGSLMNILNYPGMNHRVEITEGILADECAALLCDFYRMPRQVFNAQKKAQSSINSGGSSGGSSGSETPGTSKSAIPESSGGGSSGSAKNTITKTLKLRIVRPYNSAEVEKIVADEKNSREKIALEKNKDKVKEACSEHLKVAAYCTTQVERNACLFCKARKLDDRFYQKLRGQFPDAVFWQEIGEIFRQLQKQAAEIYNQSLIELYYEIFIKGKGFAIASSVEHYLSCVCYTRAAELFKNAAIASGLRGKVKSNFRLKELKNMKSGLPTTKSDNFPIPLVKQKGGQYTGFEISSHNDDFIIKIPFGRWQVKKEINKYRPWEKFDFEQVRKSPKPISLLLSTQRRKRNKGWSKDEGTEAEIRKVMNGDYQTSYIEVKRGSKIGEKSAWMLNLSIDVPKIDKGVDPGIIGGIDVGVKSPLVCAINNASSRYSISDNDLFHFNKKMFARRRILLKKNRHKRAGHGAKNKLKPITIMTERSKRFRKKLIERWACEIADFFIKNKVGTVQMENLESMKRKEDSYFNIRLRGFWPYSEMQNKIEFKLKQYGIEIRKVAPNNTSKTCSKCGHLNNYFNFEYRRKNKFPHFKCEKCNFKEDADYNAALNISNPKLKSTKGEP

SEQ ID NO: 1455 - protein, 726 aa, synthetic construct
SEVEFSHEYWMRHALTLAKRARDECEVPVGAILVLNNRVIGEGWNRAIGLHDPTAHAEIMALRQGGLVMQNYRLIDATLYVTFEPCVMCAGAMIHSRIGRVVFGVRNSKRGAAGSLMNVLNYPGMNHRVEITEGILADECAALLCDYYRMPRQVFNARKKAQSSINSGGSSDGGSGSETPGTSESATPESSGGSSGGSAKNTITKTLKLRIVRPYNSAEVEKIVADEKNNREKIALEKNKDKVKEACSEHLKVAAYCTTQVERSACLFCKARKLDDKFYQELRGQFPDAVFWQEIGEIFRQLQKQAAEVYNQSLVELYYEILIKGKGIANASSVEHYLSDVCYTRAAELFKNAAIASGLRNKIKSNFRLKELRNMKSGLPTTKSDNFPIPLVKQKGGQYTGFEISNHDGDFIIKIPFGRWQVKKEINKHRPWEKFDFEQVRKSPKPISLLLSTQRRKRNKGWSKDEGTEAEIRKVMNGDYQTSYIEVKRGSKIGEKSAWMLNLSIDVPKIDKGVDPSIIGGIDVGVKSPLVCAINDAFSRYSISDNDLFRFNKKVFARRRILLKKNRHKRAGHGTKNKLKPITILTEKSGRFRKKLIERWACEIADFFIKNKVGTVQMENLESMKRREDSYFNIRLRGFWPYAEMQNKIEFKLKQYGIKIRKVAPNNTSKTCSKCGHLNNYFSFEYRKKNKFPHFKCEKCNFKEDADYNAALNISNPKLKSTKEEP

SEQ ID NO: 1456 - protein, 726 aa, synthetic construct
SEVEFSHEYWMRHALTLAKRARDEREVPVGAVLVLNNRVIGEGWNRAIGLHDPTAHAEIMALRQGGLVMQNYRLTDATLYVTFEPCVMCAGAMIHSRIGRVVFGVRNSKRGAAGSLMNVLSYPGMNHCVEITEGILVDECAALLCDFYRMPRQVLNAQKKAQSSINSGGSSSGSSGSETPGTSESATPESSGGGSSGSAKNTITKTLQLRIVRPYNSAEVEKIVADEKDNRERIALEKNKGKVKEACSKHLKVAAYCTTQVERNACLFCKARKLDDKFYQKLRGQFPDAVFWQEIGEIFRQLQKQAAEIYNQSLIELYYEIFIKGKGLANASSVEHYLSDVCYTRAAELFKNAAIASGLRGKVKSNFRLKELKSMKSGLPTTKSDNFPIPLVKQKGGQYTGFEISSHNDDFIIKIPFGRWQVKKEIDKYRPWEKFDFEQVRKSPKPISLLLSTQRRKRNKGWSKDEGTEAEIRKVMNGDYRTSYIEVKRGSKTGEKSAWMLNLSIDVPKIDKGVDPSIIGGIDVGVKSPLVCAINNAFSRYSISDNDLFRFNKKMFARRRILLKKNRHKRAGHGAKNKLKPISTLTGKSERFRRKLIERWACEIADFFIKNKVGTVQMENLESMKRKEDSYFNIRLRGFWPYAEMQNKIEFKLKQYGIEIRKVAPNNTSKTCSKCGHLNNYFNFEYRKKNKFPHFKCEKCNFKEDADYNAALNISNPKLKSTKGEP

SEQ ID NO: 1457 - protein, 726 aa, synthetic construct
SEVEFSHEYWMRHALTLAKRARDEREVPVGAILVLNNRVIGEGWNRAIGLHDPTAHAEIMALRQGGLVMQNYRLTDATLYATFEPCVMCAGAMIHSRIGRVVFGVRNSKHGAAGSLMNVLNYPGMNHRVEITEGILADECAGLLCDFYRMPRQVFSARKKAQSSINPGGSSGGSSGGKAPGTSESATLESSGGSSGGSAKNSITKTLKLRIVRPYNSAEVEKIVADEKNNREKTALEKNKGKVKEACSKHLKVAAYCTTQVERNACLFCRARRLDDKFYQKLRGQFPDAVFWQEIGEIFRQLQKQAAEIYNQSLVELYYEIFIKGKGIANASGVEHYLSDVCYTRAAELFKNAAIASGLRNKIKSNFRLKELRNMKSGLPTTKSDNFPIPLVRQKGGRYTGFEISNHNSDFIIKIPFGRWQVKKEIDKYRPWEKFDFAQVRKSPKPISLLLSTQRRKRNKGWSNDEGTEAEIRKVMNGDYQTSYIEVKRGSKIGEKSAWMLSLSIDVPKIDKGVDPSIIGGIDVGVKSPLVCAINNAFSRYSISDNDLFRFNKKMFARRRILLKKNRHKRAGHGAKNKLKPISILTGKSEMFRKKLIERWACEIADFFIKNKVGTVQMENLESMKRREDSYFNIRLRGFWPYAEMQNKIEFKLKQYGIEIRKVAPNNTSKTCSKCGHLNNYFNFEYRKKNKFPHFKCEKCNFKENADYNAALNISNPKLKSTKEEP

SEQ ID NO: 1458 - protein, 726 aa, synthetic construct
SEVEFSHEYWMRHALTLAKRARDEREVPVGAVLVLNNRVIGEGWNRAIGLHDPTAHAEIMALRQGGLVTQNYRLIDATLYVTFEPCVMCAGAMIHSRIGRVVFGVRNNKHGAAGSLVNVLNYPGMNHRVEITEGILADECAALLCDFYRMPRQVFNARKRAQSSISPGGSSGGSSGSETPGASESVTPKSSGGSSGGSAKNTITKTLQLRIVRPYNSAEVEKIVADEKNNREKIALEKNKDKVKEACSKHLKVAAYCTTQVERNACLFCKARKLDDKFYQKLRGQFPDAVFWQEIGEIFRQLQKQAAEIYNQSLIELYYEIFIKGKGFANASSVEHYLSDVCYTRAAELFKNAAIASGLRGKVKSNFRLKELKNMKSGLPTTKSDNFPIPLVKQKGGQYTGFEISSHNDDFIIKIPFGRWQVKEEIDKYRPWEKFDFEQVRKNPKPISLLLSTQRRKRNKGWSKDEGTEAEIRKVMNGDYQTSYIEVKRGSKIGEKSAWMLNLSIDVPKIDKGVDPSIIGGIDVGVKSPLVCAINNALSRYSISDNDLFHFNKKMFARRRILLRKNRHKRAGHGARNKLKPITVLTEKSERFRKKLIERWACEIANFFIKNKVGTVQMENLESMKRREDSYFNIRLRGFWPYAEMQNKIEFKLKQYGIKIRKVAPNNTSKTCSKCGHLNNYFSFEYRKKNKFPHFKCEKCNFKEDADYNAALNISNPKLKGTKEEP

SEQ ID NO: 1459 - protein, 726 aa, synthetic construct
SEVEFSHEYWMRHALTLAKRARDEREVPVGAVLVLNNRVIGEGWNRAIGLHDPTAHAEIMALRQGGLAMQNYRLVDATLYVTFEPCVLCAGAMVHSRIGRVVFGVRNSKRGAAGSLMNVLNHPGMNHRVEITGGILADECAALLCDFYRMPRRVFNAQKKARSNINSGGSSGGSSGSEAPGTSESATPESSGGSSGGSAKNTITKTLQLRIVRPYNSAEVEKIVADEKNNREKIALEKNKDKVKEACSQHLKMASYCTTQVERNACLFCKARKLDDKFYQKLRGQFPDAVFWQEIGEIFRQLQKQAAEIYNQSLIELYYEIFIKGKGFANASSVEHYLSDVCYTRAAELFKNAAIASGLRGKVKSNFRLKELKNMKSGLPTTKSDNFPIPLVKQKGGQYTGFEVSSHNDDFIIKIPFGRWQVKKEIDKYRPWEKFDFEQVRKSPKPISLLLSTQRRKRNKGWSKDEGTEAEIKRVMNGDYQTSYIEVKRGSKIGEKSAWMLNLSIDVPKIDKGVDPSIIGGIDVGVKSPLVCAINNAFGRYSISDNDLFHFNKKMFARRRILLKRNRHKRAGHGAKNKLKPITILTEKSKRFRRKLIERWACEIADFFIKNKVGTVQMENLESMKRKEDSYFNIRLRGFWPYAEMQDKIEFKLKQYGIEIRKVAPNNTSKTCSRCGHLNNYFNFEYRRKNKFPHFKCEKCNFKENADYNAALNISNPKLKSTKEEP

SEQ ID NO: 1460 - protein, 726 aa, synthetic construct
SEVEFSHEYWMRHALALAKRARDEREVPVGAILVLNNRVIGEGWNRAIGLHDPTAHAEIMALRQGGLVMRNYRLTDATLYVTFEPCVMCAGAMIHSRIGRVVFGVRNSKHGAAGSLMNVLNYPGMNHRVEITEGVLADECAALLCDFYRMPRQVFSARKKAQSSINPGGSSGGSSGSKTPGTSESATPESSGGSSGGSAKNSITKTLKLRIVRPYNSAEVEKIVADEKNNREKIALEKNKGKVKEACSKHLKVATYCTTQVERNACLFCKARKLDDKFYQKLRGQFPDAVFWQEIGEIFRQLQKQAAEIYNQSLIELYYEIFIKGKGITNASRVEHYLSDVCYTRAAELFKNAAIASGLRSKVRSNFRLKELKNMRSGLPTTKSDNFPIPLVKQKGGQHTGFEISSHNSDFIIKIPFGRWQVKEGIDKYRPWEKFDFEQVRKSPKPISLLLSTQRRKKNKGWSKDEGTEAEIRRVMNGDYQTSYIEVKRGSKIGEKSAWMLNLSIDVPKIDKGVDPSIIGGIDVGVKSPLVCAVNNSFSRYSICDNDLFRFNKKMFARRRILLKKNRHKRAGHGAKNKLKPITILTKKSERFRRKLIERWACEVADFFIKNKVGTVQMENLESMKRKEDSYFNIRLRGFWPYAEMQNKIEFKLKQYGIETRKVAPNNTSKTCSKCGHLNNYFSFEYRKKNKFPHFKCEKCNFKEDADYNAALNISNPKLKSTKEEP

SEQ ID NO: 1461 - protein, 726 aa, synthetic construct
SEVEFSHEYWMRHALTLAKRARDEREVPVGAVLVLNNRVIGEGWNRTTGLHDPTAHAEIMALRQGGLVMQNHRLVDATLYVTFEPCVMCAGAMIHSRIGRVVFGVRNSKRGAAGSLTNVLNYPGMNHRVEITEGILVDECAALLCDFYRMPRQVFNAQKKAQSTINSGGSSGGSSGSETPGTSESATPESSGGSSGGSAKNTITKTLTLRIVRPYNSAEVEKIVADEKNNREKIALEKNRDKVKEACSKHLKVAAYCTTQVERNACLFCKARKLDDRFYQKLRGQFPDAVFWQEIGEIFRQLQKQAAEIYNQSLIELYYEIFIKGKGFANASSVEHYLSDVCYARAAELFKNAAIASGLRGKVKSNFRLKELKNMRSGLPTTKSDNFPIPLVKQKGGQYTGFEISSHNDDFIIKIPFGRWQVKKEIDKYRPWEKFDFEQVRKSPKPISLLLSTQRRKRNKGWSKDEGTEAEIRKVMNGDYQTSYIEVKRGSKIGEKSAWMLNLSIDVPKIDKGVDPSIIGGIDVGVKSPLVCAINNALGRYSISDNDLFHFNKKMFARRRILLKKSKHKRAGHGAKNKLKPITILTEKSGRFRKKLIERWACEIADFFIKNKVGTVQMENLESMKRREDSYFNIRLRGFWPYAEMQNKIEFKLKQYGIEIRKVAPNNTSKTCSKCGHLNNYFNFEYRKMNKFPHFKCEKCNFKENADYNAALNISNPKLKSTKEEP

SEQ ID NO: 1462 - protein, 726 aa, synthetic construct
SEVEFSHEYWMRHALTLAKRARDEREVPVGAVLVLNNRVIGAGWNRTTGLHDPTAHAEIMALRQGGLVMQNHRLVDATLYVTFEPCVMCAGAMIHSRIGRVVFGIRNSKRGAAGSLTNVLDYPGMSHRVEITEGILADECAALLCDFYRMPRQVFNAQKKAQSNINPGSSSGGSSGSETPGTSESATPGSSGGSSGGSAKNTITKTLKLRIVRPYNSAEVEKIVADEKNNREKIALEKNKDKVKEACSKHLKVAAYCTTQVERNACLFCKARRLDDKFYQKLRGQFPDAVFWQEIGEIFRQLQKQAAEIYNQSLIELYYEIFIKGKGFANASSVEHYLSDVCYTRAAELFKNAAIASGLRGKVKSNFRLKELKNMKSGLPTTKSDNFPIPLVKQKGGQYTGFEISSHNDDFIIKIPFGRWQVKKEIDKYRPWEKFDFEQVRKSPKPISLLLSTQRRKRNKGWSKDEGTEAEIRKVMNGDYQTSYIEVKRGSKIGEKSAWMLSLSIDVPKIDKDVDPSIIGGIDVGVRSPLVCAINNAFSRYSISDNDLFHFNKKIFARRRILLKKNRHKRAGHGAKNKLKPITILTEKSVRFRKKLIERWACEIADFFIKNKVGTVQMENLESMKRKEDSYFNIKLRGFWPYAEMQNKIEFKLKQYGIEIRRVAPNNTSKTCSKCGHLNNYFNFEYRKKNKFPHFKCEKCSFKENADYNAALNVSNPKLKSTKEEP

SEQ ID NO: 1463 - protein, 726 aa, synthetic construct
SEVEFSHEYWMRHALSLAKRARDEREVPVGAVLVLNNRIIGEGWNRAIGLHDPTAHAEIMALRQGGLVMQNYRLTDATLYVTFEPCVMCAGAMVHSRIGRVVFGVRNSKRGAAGSLMNVLNYPGVSHCVEITEGILVDECAALLCDFYSMPRQVLNAQKRAQSSINSGGSSGGSSGSETPGTSGSATPGSSGGGSSGSAKNTITKTLQLRIVRPYNSAEVEKIVADEKNNREKIALEKNKDKVKEACSKHLKVASYCTTQVERNACLFCKARKLDDKFYQKLRGQFPDAVFWQELGEIFRQLQKQAAEIYNRSLIELYYVIFIKGKGFANASSVEHYLSDVCYTRAAELFKNAAIASGLRGKVKSNFRLKELKNMKSGLPTTKSDNFPIPLVKQKGGQYTGFEISSHNDDFIIKVPFGRWQVKKEIDKYRPWEKFDFEQVRKSPKPISLLLSTQRRKRNKGWSKDVGTEAEIRKVMNGDYQTSYIEVKRGSKIGEKSAWMLNLSIDVPKIDKGVDPSIVGGIDVGVKSPLVCAIDNALSRYSISDNDLFHFNKKMFARRRVLLKKNRHRRAGHGVKNKLKPISILTEKSKRFRKKLIERWACEIADFFIKNKVGTVQMENLESMKRKEDSYFNIRLRGFWPYAEMQNKIEFKLKQYGIEVRKVAPNNTSKTCSRCGHLNNYFNFEYRKKNKFPHFKCEKCNFKEDADYNAALNISNPKLKSTKEEP

SEQ ID NO: 1464 - protein, 726 aa, synthetic construct
SEDEFSHEYWMRHALTLAKRARDGREVPVGAVLVLNNRVIGEGWNRAIGLHDPTAHAEIMALRQGGLVMQNYRLIDATLYVTFEPCVMCAGAMVHSRIGRVVFGVRNSKRGAAGSLMNVLDYPGMGHRVEITEGILADECAALLCDFYCMPRQVFNAQKRVQSSINSGGSSGGSSGSETPGTSESATPERSGGGSSGSAKNTITKTLQLRIVRPYNSAEVEKIVADEKNNREKIALEKNKDKVKEACSKHLKVASYCTTQVERNACPFCKARKLDDKFYQKLRGQFPDAVFWQELGEIFRQLQKQAAEIYNQSLIELYYEIFIKGRGFANASSVEHYLSDVCYTRAAELFKNAAIASGLRGKVKSNFRLKELKNMRSGLPTTKSDNFPIPLVKQKGGQYTGFEISSHNDDFIIKIPFGRWQVKKEIDKYRPWEKFDFERVRKSPKPISLLLSTQRRKRNKGWSKDEGTEAEIRKVMNGDYQTSYIEVKRGSKIGEKSAWMLSLSIDVPKIDKGVDPSVIGGIDVGVKSPLVCAINNAFCRYSISDNDLFHFNKKMFARRRILLKKSRHKRAGHGAKNKLKPISILTEKSKRFRKKLVERWACEIADFFIKNKVGTVQMENLESMKRKEDSYFNIRLRGFWPYAEMQNKIEFKLKQYGIEIRKVAPNNTSKTCSKCGHLNNYFNFEYRKKNKFPHFKCEKCNFKENADYNAALNISNPKLKSTKEKP

SEQ ID NO: 1465 - protein, 726 aa, synthetic construct
SGVEFSHEYWMRHALTLAERARDGHEVPVGAVLVLNNRVIGEGWNRAIGLNDPTAHAEIMALRQGGQVMQNYRLIDATLYVTFEPCVMCAGAMVHSRIGRVVFGVRNSKRGAAGSLMNVLDYPGMDHRVKITEGILADECAALLCDFYRMPRQVFNAQKKAQSSINSGGSSGGSSGSETPGTSESATPESSGGSSGGSAKNTITKTLKLRIVRPYNSAEVEKIVADEKNNREKIALEKNKDKVKEACSEHLKVAAYCTTQVERNACLFCRARRLDDKFYQKLRGQFPDAVFWQELGEILRQLQKQAAEIYNQSLIELYYEIFIKGRGFANASSVEHYLSDVCYTRAAELFKNAAIASGLRGKVKSNFRLKELKNMKSGLPTTKSDNFPIPLVKQKGGQYTGFEISNHNGDFIIKIPFGRWQVKKEIDKYRPWEKFDFEQVRKSPKPISLLLSTQRRKRNKGWSKDEGTEAEIRKVMNGVYQTSYIEVKRGSKTGEKSAWMLNLSIDVPKIDKGVDPSIIGGIDVGVKSPLVCAINNAFSRYSISDNDLYRFNKKMFARRRILLKKSKHKRAGHGAKNKLKPITILTEKSGRFRKKLIERWACEIADFFIKNKVGTVQMENLEGMKRREDSYFNIRLRGFWPYAEMQNKIEFKLKQYGIEIRKVAPNNTSKTCSKCGHLNNYFNFEYRKKNKFPHFKCEKCNFKENADYNAALNISNPKLKSTKEEP

SEQ ID NO: 1466 - protein, 726 aa, synthetic construct
SEVEFSHEYWMRHALTLAKRARDEREVPVGAVLVLNNRVIGEGWNRAIGLHDPTAHAEIMALRQGGLAMQNYRLVDATLYVTFEPCVLCAGAMVHSRIGRVVFGVRNSKRGAAGSLMNVLNYPGMNHRVEITEGILADECAALLCDFYRMPRQVFNAQKKARSNINSGGSSGGSNGSETPGTSESATPGSSGGSSGGSAKNTITKTLKLRIVRPYNSAEVEKIVADEKNSREKIALERNKDKVKEACSEHLKVAAYCTTQVERNACLFCKARKLDDRFYQKLRGQFPDAVFWQETGEIFRQLQRQAAEIYNQSLIELYYEIFIKGKGFANASSVEHYLSDVCYTRAAELFKNAAIASGLRGKVKSNFRLKELKNMKSGLPTTKSDNFPIPLVKQKGGQYTGFEISSHNDDFIIKIPFGRWQMKKEIDRYRPWEKFDFEQVRKSPKPISLLLSTQRRKRNKGWSKDEGTEAEIRKVMNGDYQTSYIEVKRGSKIGEKSAWMLSLSIDVPKIDKGVDPSIIGGIDVGVKSPLVCAINNALSRYSISDNDLFHFNKKMFARRRILLRKNRHKRAGHGARNKLKPITVLTEKSERFRKKLIERWACEIANFFIKNKVGTVQMENLESMKRREDSYFNIRLRGFWPYAEMQSKIEFKLKQYGIKIRKVAPNNTSKTCSKCGHLNNYFNFEFRKKNKFPHFKCEKCNFKEDADYNAALNISNPKLKGTKEEP

SEQ ID NO: 1467 - protein, 726 aa, synthetic construct
SEVEFSHEYWMRHALTLAKRARDEREVPVGAVLVLNNRVIGGGWNRAIGLHDPTAHAEIMALRQGGLVTQNYRLVDATLYVTFEPCVMCAGAMIHSRIGRVVFGVRNSKRGAAGSLMNVLNYPGMNHCVEITEGILVDECAALLCDFYRMPRQVLNAQKKAQTSISPGGSSGGSSGSETPGASGSVTPKSSGGSSAGSTKDTITKTLKLRIVRPYNSAEVEKIVADEKNNREKIALEKNKDKVKEACSKHLKVAAYCTTRVERNACLFCKARRLDDKFYQKLRSQFPDAVFWQEIGEIFRQLQKQAAEIYNQSLIELYYEIFIKGKGFANASSVEHYLSDVCYTRAAELFKNAAIASGLRGKVKSNFRLKELKNMRSGLPTTKSDNFPIPLVKQKGGQYAGFEISSHNDDFIIKIPFGRWQVKKEIDKYRPWEKFDFEQVRKSPKPISLLLSTRRRKRNKGWSKDEGTEAEIRKVMNGDYQTSYIEVKRGSKIGEKSAWMLNLSIDVPKIDKGVDPSIIGGIDVGVKSPLVCAINNALSRYSISDNDLFHFNKKMFARRRILLRKNRHKRAGHGARNKLKPITVLTEKSERFRKKLIERWACEIADFFIKNKVGTVQMENLESMKRKEDSYFNIRLRGFWPYAEMQNKIEFKLKQYGIVVRKVAPNNTSKTCSKCGHLNNHFNFEYRKKNKFPHFKCKKCNFKEDADYNAALNISNPKLESTKGEP

SEQ ID NO: 1468 - protein, 726 aa, synthetic construct
SEVEFSHEYWMRHALTLAKRARDEREVPVGAVLVLNNRVIGEGWNRTTGLHDPTAHAEIMALRQGGLVMRNYRLTDATLYVTFEPCVMCAGAMIHSRIGRVVFGVRNSKRGAAGSLMNVLNYPGMNHRVEITEGILADECAALLCDFYRMPRQVFNARKKAQSSINPGSLSGGSSGGETPGTSESATPESSGGSSGGSAKNTITKTLKLRIVRPYNSAEVEKIVADEKNNREKIALEKNKDKVKEACSEHLKVAAYCTTQVERSACLFCKARKLDDKFYQKLRGQFPDAVFWQEIGEIFRQLQKQAAEIYNQSLIELYYEIFIKGKGFANASSVEHYLSDVCYTRAAELFKNAAIASGLRGKVKGNFRLKELKNMKSGLPTTKSDNFPIPLVKQKGGQYTGFEISSHNDDFIITIPFGRWQVKKEIDKYRPWEKFDFAQVRKSPKPISLLLSTQRRKRNKGWSKDEGTEAEIRKVMNGDYQTSYIEVKRGSKTGEKSAWMLNLSIDVPKIDKGVDPSIIGGIDVGVKSPLVCAINNAFSRYSISDNDLFHFNKKMFARRRILLKKNRHRRAGHGAKNKLKPITILTEKSVRFRRKLIERWACEIADFFVKNKVGTVQMENLESMKRKEDSYFNIRLRGFWPYAEMQNKIEFKLKQYGIEIRKVAPNNTSRTCSKCGHLNGYFNFEYRKKNKFPHFKCEKCSFKENADYNAALNISNPKLKSTKEEP

SEQ ID NO: 1469 - protein, 726 aa, synthetic construct
SEVEFSHEYWMRHALTLAKRARDEREVPVGAILVLNNRVIGEGWNRAIGLHDPTAHAEIMALRQGGLVMQNYRLTDATLYATFEPCVMCAGAMIHSRIGRVVFGVRNSKHGAAGSLVNVLNYPGMNHRVEITEGILANECAALLCDFYRMPRQVFNARKKAQSSINPGGSSGGSSGSETPGTSESATPKSSGGSSAGSTKSTITKTLKLRIVRPYNSAEVEKIVADEKNSREKIALEKNKDKVKEACSKHLKVAAYCTTQVERNACLFCKARKLDDKFYQKLRGQFPDAVFWQEIGEVFRQLQKQAAEIYNQSLIELYYEIFIKGKGFANASSVEHYLSDVCYTRAAELFKNAAIASGLRGKVKSNFRLKELKNMKSGLPTTKSDNFPIPLVKQKGGQYTGFEISSHDDDFVIKIPFGRWQVKEEIDKYRPWEKFDFEQVRKNPKPISLLLSTRRRKGNKGWSKDEGTEAEIRKVMNGDYQTSYIEVKRGSKIGEKSAWMLNLSIDVPKIDKGVDPSIIGGIDVGVKSPLVCAINNAFSRYSISDNDLFRFNKKMFARRRILLKKNRHKRTGHGAKNKLKPISILTEKSGRFRKKLIERWACEIADFFVKNKVGTVQMENLESMKRKEDSYFNIRLRGFWPYAEMQNKIEFKLKQYGIKVRKVAPNNTSKTCSKCGHLNNYFSFEYRKKNKFPHFKCEKCNLKENADYNAALNISNPKLKSTKEEP

SEQ ID NO: 1470 - protein, 726 aa, synthetic construct
SEVEFSHEYWMRHALTLAKRARDEREVPVGAILVLNNRVIGEGWNRAIGLHDPTAHAEIMALRQGGLVMQNYRLIDATLYVTFEPCVMCAGAMIHSRIGRVVFGVRNNKHGAAGSLMNVLNYPGMNHCVEITEGILVDECAALLCDFYRMPRQVFNAQKKAQSTINSGGSSGGSSGSETPGTSESPTPESSGGSPGGSAKNTITKTLKLRIVRPYNSAEVEKIVADEKDNREKIALEKNKDKVKGACSKHLKVASYCTTQVERNACPFCKARKLDDKFYQKLRGQFPDAVFWQELGEILRQLQKQAAEIYNQSLIELYYEIFIKGKGLANASSVEHYLSDVCYTRAAELFKNAAIASGLRGKVKSNFKLKELKSMKSGLPSTKSDNFPIPLVKQKGGQYTGFEISSHNDDFIIKIPFGRWQAKKEIDKYRPWEKFDFEQVRKSAKPISLLLSTQRRKRNKGWSKDEGTEAEIRKVMNGDYQTSYIEVKRGSKIGEKSAWMLNLSIDVPKIDKGVDPSIIGGIDVGVKSPLVCAINNAFSRYSISDNDLFHFNKKMFARRRILLKKNRHKRAGHGAKNKLKPISILTEKSKRFRKKLIERWACEIADFFIKNKVGTVQMENLESMKRKEDSYFNIRLRGFWPYAEMQNKIEFKLKQYGIGIRKVAPNNTSKTCSKCGHLNNYFNFEYRRKNKFPHFKCEKCNFREDADYNAALNISNPKLKSTKEEP

SEQ ID NO: 1471 - protein, 726 aa, synthetic construct
SEVEFSHEYWMRHALTLARRARDEREVPVGAILVLNNRVIGEGWNRAIGLHDPTAHAEIMALRQGGLVMQNYRLINATLYVTFEPCVMCAGAMIHSRIGSVVFGVRNSKHGAAGSLMNVLNYPGMNHRVEITEGILADECAALLCDFYRMPRQVFNAQKKAQSSINSGGSSSGSSGSETPSTCESATPESSGGGSSGSAKNTITKTLQLRIVRPYNSAEVEKIVADEKNNREKIALEKNKDKVREACNKHLKVASYCTTQVERNACPFCKARKLDDKFYQKLRGQFPDAVFWQELGEILRQLQKQAAEIYNQSLIELYYEIFIKGRGFANASSVEHYLSDVCYTRAAELFKNAAIASGLRGKVKSNFRLKELKNMKSGLPTTKSDNFPIPLVKQKGGQYTGFEISNHNGDFIIKIPFGRWQVKKEISKHRPWEKFDFEQVRKSPKPISLLLSTQRRKRNKGWGKDEGTEAEIRKVMNGDYQTSYIEVKRGSKTGEKSAWMLNLSIDVPKIDKGVDPSIIGGIDVGVKSPLVCAINNAFSRYSISDNDLFRFNKKMFARRRILLKKNRHKRAGHGAKNKLKSISILTGKSERFRKKLIERWACEIADFFIKNKVGTVQMENLESMKRKEDSYFNIRLRGFWPYAEMQNKIEFKLKQYGIEIRKVAPNNTSKTCSKCGHLNNYFNFEYRKKNKFPHFKCEKCNFKENADYNAALNISNPKLKSTREEP

SEQ ID NO: 1472 - protein, 726 aa, synthetic construct
SEVEFSHEYWMRHALTLAKRARDEREVPVGAVLVLNNRVIGEGWNRAIGLHDPTAHAEIMALRQGGLVMQNCRLVDATLYVTFEPCVMCAGAMVHSRIGRVVFGVRNSKRGAAGSLMNVLNYPGMNHRVEITEGILADECAALLCDFYRMPRQVFNARKKARSNINSGGSSGGSSGSETPGTSESATPESSGGSSGGSAKNTITKTLKLRIVRPYNSAEVEKIVADEKNNREKIALEKNKDKVKEACSEHLKVAAYCTTQVERNACLFCKARKLDDKFYQKLRGQFPDAVFWQEISEIFRQLQKQAAEIYNQSLIELYYEIFIKGKGFANASSVEHYLSDVCYTRAAELFKNAAIASGLRGKVKSNFRLKELKNMKSGLPTTKSDNFPIPLVKQKGGQYTGFEISSHNDDFIIKIPFGRWQVKKEIDKYRPWEKFNFEQVRKSPKPISLLLSTQRRKRNKGWSKDEGTEAEIRKVMNGDYQTSYIEVKRGSKIGEKSVWMLSLSIDVPKIDKGVDPSIIGGIDVGVKSPLVCAINNAFNRYSISDNNLFHFNKKMFARRRILLKKNRHKRAGHGAKNKLKPITILTEKSKRFRKKLIERWACEIADFFIKNKVGTVQMENLESMKRKEDSYFNTRLRGFWPYAEMQSKIEFKLKQYGIEIRKVAPNNTSKTCSKCGHLNNYFSFEYRKRNKFPHFKCEKCNFKENADYNAALNISNPKLKGTKEEP

SEQ ID NO: 1473 - protein, 726 aa, synthetic construct
SEVEFSHEYWMRRALTLAKRARDEREVPVGAVLVLNNRVIGVGWNRAVGLHDPTAHAEIMALRQGGLVMQNYRLIEATLYVTFEPCIMCAGAMIHSRIGRVVFGVRNSKRGAAGSLMNVLNYPGMNHRVEITEGILADECAALICDYYRMPRQVFNARKKVQSSINSGGSSDGGSGGETPGTSESATPESSGGSSGGSAKNTITKTLKLRIVRPYNSAEVEKIVADEKNNREKIALEKNKDKVKEACSEHLKVAAYCTTQVERNACLFCKARKLDDKFYQKLRGQFPDAVFWQELGEIFRQLQKQAAEIYNQSLIELYYEIFIKGKGFANASSVEHYLSDVCYTRAAELFKNAAIASGLRGKVKSNFRLKELKNMKSGLPTTKSDNFPIPLVKQKGGQYTGFEISSHNDDFIIKIPFGRWQVRKEIDKYRPWERFDFEQVRKSPKPISLLLSTQRRKRNRGWSKDEGTEAEIRKVMNGDYQTSYIEVKRGSKTGEKSAWMLNLSIDVPKIDKGVDPSIIGGIDVGVKSPLVCAINNSSSRYSICDNDLFRFNKKMFARRRILLKKNRHKRAGHGAKNKLKPITILTERSKRFRKKLIERWACEIADFFIKNKVGTVQMENLESMKRKEDSYFNIRLRGFWPYAEMQNKIEFKLKQYGIEIRKVAPNNTSRTCSKCGHLNNYFNFEYRKENKFPHFKCEKCNFKEDADYNAALNISNPKLKSTKEEP

SEQ ID NO: 1474 - protein, 726 aa, synthetic construct
SEVEFSHEYWMRHALTLAKRARDEREVPVGAILVLNNRVIGEGWNRAIGLHDPTAHAEIMALRQGGLVMQHYRLIDATLYVTFEPCVMCAGAMIHSRIGRVVFGVRNSKHGAAGSLMNVLNYPGMNHRVEITEGILADECAALLCDFYRMPHQVFNARKKAQSSINPGGPSGGSSGSETPDTSESATPESSGGSSGGSAKNTITKTLKLRIVRPYNSAEVERIVADEKNSREKIALEKNKDKVKEACSKHLRVAAYCTTQVERNACLFCKARKLDDKFYQRLRGQFPDAVFWQELGEIFRQLQKQAAEIYNQSLIELYYEIFIKGKGFANASSVEHYLSDVCYTRAAELFKNAAIASGLRGKVKSNFRLKELKNMKSGLPTTKSDNFPIPLVKQKGGQYTGFEISSHNDDFIIKIPFGRWQVKKEIDKYRPWEKVDFEQVRKSPKPISLLLSTQRRKRNKGWSKDEGTEAEIRKVMNGDYQTSYIEVKRGSKIGEKSAWMLNLSIDVPKIDKGVDPSIIGGIDVGVKSPLVCAINNALSRYSISDNDLFRFNKKMFARRRILLKKNRHKRAGHGAKNKLKPISILTGKSERFRKKLIERWACEIADFFIKNKVGTVQMENLESMKRKEDSYFNIRLRGFWPYAEMQNKIEFKLKQYGIEIRKVAPNNTSKTCSKCGHLNNYFNFEYRKKNKFPHFKCEKCNFKENADYNAALNISNPKLKSTKEEP

SEQ ID NO: 1475 - protein, 726 aa, synthetic construct
SEVEFSHEYWMRHALALAKRARDEREVPVGAVLVLNNRAIGEGWNRAIGLHDPTAHAEIMALRQGGLVMQNYRLTDATLYVTFEPCVMCAGAMIHSRIGRVVFGVRNSKRGAAGSLMNVLNYPGMNHCVEITEGILVDECAALLCDFYRMPRQVLNAQKKAQSSINSGGSSDGGSGSETPGTSESATPESSGGSSGGSAKNTITKTLKLRIVRPYNSAEVEKIVADEKNNREKIALEKNKDKVKEACSKHLKVAAYCTTQVERNACLFCKARKLDDKFYQKLRGQFPDAVFWQEISEILRQLQKQAAEIYNQSLIELYYEIFIKGKGFANASSVEHYLSDVCYTRAAELFKNAAIASGLRGKVKSNFRLKELKNMKSGLPTTKSGNFPIPLVKQKGGQYTGFEISSHNDDLIIKIPFGRWQVKKEIDRYKPWEKFDFEQVRKSPKPISLLLSTQRRKRNKGWSKDEGTEAEIRKVMNGDYQVSYIEVKRGSRIGEKSAWMLSLSIDVPKIDKGVDPSIIGGIDVGVKSPLVCAINNALSRYSISDNDLFHFNKKMFARRRILLKKNRHKRNGHGARNKLKPITVLAEKSERFRKKLIERWACEIANFFIKNKVGTVQMENLESMKRKEDSYFNIRLRGFWPYAEMQNKIEFKLKQYGIKIRKVAPNNTSKTCSKCGHLNNYFSFEYRKKNKFPHFKCEKCNFKENADYNAALNISNPKLKSTKEEP

SEQ ID NO: 1476 - protein, 726 aa, synthetic construct
SEVEFSHEYWMRHALTLAKRARDEREVPVGAVLVLNNRVIGEGWNRTTGLHDPTAHAEIMALRQGGLVMQNHRLVGATLYVTFEPCVMCAGAMIHSRIGRVVFGVRNGKRGAAGSLTNVLNYPGMNHRVEITEGILVDECAALLCDFYRMPRQVFNAQKKAQSTINSGGSSGGSSGSETPGTSESPTPESSGGSPGGSAKNTITKTLKLRIVRPYNSAEVEKIVADEKNNREKIALEKNKDKVKEACSKHLKVASYCTTQVERNACLFCKARKLDDKFYQKLRGQFPDAVFWQEISEIFRQLQKQAAEIYNQSLIELYYEIFIKGKGFANASSVEHYLSDVCYTRAAELFKNAAIASGLRGKVKSNFRLKELKNMKSGLPTTKSDNFPIPLVKQKGGQYTGFEISSHNDDFIIKIPFGRWQVKKEVDKYRPWEKFDFEQVRKSPKPISLLLSTQRRKKNKGWSKDEGTEAEIRRVMNGDYQTSYIEVKRGSKIGEKSAWMLSLSIDVPKIDKGVDPSIIGGIDVGVKSPLVCAINNAFSRYSISDNDLFRFNKKMFARRRILLRKNRHRRAGHGAKNKLKPITILTEKSERFRKKLVEKWACEIADFFIKNKVGTVQMENLESMKRREDSYFNIRLRGFWPYAEMQNKIEFKLKQYGIEIRRVAPNNTSKTCSKCGHLNNYFNFEYRKKNKFPHFKCEKCNFKENADYNAALNISNPKLKSTKEEP

SEQ ID NO: 1477 - protein, 726 aa, synthetic construct
SEVEFSHEYWMRHALTLAKRARDEREVPVGAILVLNNRVIGEGWNRAIGLHDPTAHAEIMALRQGGLVMQNHRLIDATLYVTFEPCVMCAGAMIHSRIGRVVFGVRNNKHGAAGSLVNVLNYPGMNHRVEITEGILADECAALLCDFYRMPRQVFNARKKARSNINSGGSSGGSSGSEAPGTSESATPESSGGSSGGSTRNTITKTLKLRIVRPYNSAEVEKIVADEKNSREKIALERNKDKVKEACSEHLKVAAYCTTQVERNACLFCKARKLDDRFYQKLRGQFPDAVFWQETGEIFRQLQRQAAEIYNQSLIELYYEIFIKGKGFANASSVEHYLSDVCYTRAAELFKNAAIASGLRGKVKSNFRLKELKNMRSGLPTTKSDNFPIPLVKQKGGQYTGFEISSHNDDFIIKIPFGRWQVKKEIDKYRPWEKFDFEQVRKSPKPISLLLSTQRRKRNKGWSKDEGTEAEIRKVMNGDYQTSYIEVKRGSKTGEKSAWMLNLSIDVPKIDKGVDPCVIGGIDVGVKSPLVCAINNAFSRYSISDNDLFRFNKKVFARRRILLKKNRHKRAGHGTKNKLKPIAILAEKSGRFRKKLIERWACEIANFFIKNKVGTVQMENLEGMKRKEDSYFNIRLRGFWPYAEMQNKIEFKLKQYGIKIRKVAPNNTSKTCSKCGHLNNYFSFEYRKKNKFPHFKCEKCNFREDADYNAALNISNPKLKSTKEDP

SEQ ID NO: 1478 - protein, 726 aa, synthetic construct
SEVEFSHEYWMRHALTLAKRARDEREVPVGAVLVLNNRVIGEGWNRAIGLHDPTAHAEIMALHQGGLVMQNYRLIDATLYVTFEPCVMCAGAMIHSRIGRVVFGARNSKRGAAGSLMNVLSYPGMNHRVEITEGILADECAALLCDFYRMPRRVFNAQKRAQSSINSGGSSGGSSGSETLGASESATPESSGGGSSGSAKNTITKTLQLRIVRPYNSAEVEKIVADEKNNREKIALEKNKDKVREACSKHLKVAPYCTTQVERNACPFCKARKLDDKFYQKLRGQFPDAVFWQEIGEIFRQLQKQAAEIYNQSLIELYYEIFIKGKGFANASSVEHYLSDVCYTRAAGLFKNAAIASGLRGKVKSNFRLKELKNAKSGLPTTKSDNFPIPLVKQKGGQYTGFEISSHNDDFIIKIPFGRWQVKEEIDKYRPWEKFDFEQVRKNPKPISLLLSTQRRKRNKGWSKDEGTEAEIRRVMNGDYQTSYIEVKRGSKIGEKSAWMLNLSIDVPKIDKGVDPSIIGGIDVGVKSPLVCAINNAFSRYSISDNDLFRFNKKVFARRRILLKKNRYKRAGHGTKNKLKPITILTEKSGRFRKKLIERWACEIANFFIKNKVGTVQMENLESMKRKEDSYFNIRLRGFWPYAEMQNKIEFKLKQYGIEIRKVAPNNTSKTCSKCGHLNSYFNFEYRKKNKFPHFKCEKCNFKENADYNAALNISNPKLKSTKEEP

SEQ ID NO: 1479 - protein, 726 aa, synthetic construct
SEVEFSHEYWMRHALTLAKRARDEREVPVGAVLVLNDRVIGEGWNRTTGLHDPTAHAEIMALRQGGLVMQNHRLVDATLYVTFEPCVMCAGAMIHSRIGRVVFGVRNSKRGAAGSLTNVLNYPGMGHRVEITEGILVDECAALLCDFYRMPRQVLNAQKKAQSSISSGGSSGGSSGSETSGASESATPKSSGGSSAGSTKNTITKTLKLRIVRPYNSAEVEKIVADEKNSRERIALEKNKDKVKEACSKHLKVAAYCTTQVERSACLFCKARKLDDKFYQELRGQFPDAVFWQEIGEIFRQLQKQAAEIYNQSLIELYYEIFIKGKGFANASSVEHYLSDVCYTRAAELFKNAAIASGLRGKVKSNFRLKELKSMKSGLPTTKSDNFPIPLVKQKGGQYTGFEISSHNDDFIIKIPFGRWQVRKEIDKYRPWEKYNFEQVRKSPKPISLLLSTQRRKRNKGWSKDEGTEAEIRKVMNGDYQTSYIEVKRGSKIGEKSAWMLSLSIDVPKIDKGVDPSIIGGIDVGVKSPLVCAINNAFNRYSISDNNLFHFNKKMFARRRILLKKNRHKRVGHGAKNKLKPISILTEKSERFRKKLIERWACEIADFFIRNKVGTVQMENLEGMKRKEDSYFNIRLRGFWPYAEMQNKIEFKLKQYGIVVRKVAPNNTSKTCSKCGHLNNYFNFEYRKKNKFPHFKCEKCNFKEDADYNAALNISNPKLKSTKGEP

SEQ ID NO: 1480 - protein, 726 aa, synthetic construct
SEVEFSHEYWMRHALTLAKRARDEREVPVGAILVLNNRVIGVGWNRAIGLHDPTAHAEIMALRQGGLVMQNYRLIDATLYVTFEPCVMCAGAMIHSRIGRVVFGVRNSKHGAAGSLVNVLNYPGMNHRVEITEGILADECAALLCDFYRMPRQVFNARKKAQSSINSGGSSGGSNGSVTPGTSESATPESSGGSFGGSAKNTVTKTLQLRIVRPYNSAEVEKIVADEKNSREKIALEKNKGKVKEACSKHLEVAAYCTTQVERNACLFCKARKLDDKFYQKLRGQFPDAVFWQELGEIFRQLQKQAAEIYNQSLIELYYEIFIKGKGFANASSVEHYLSDVCYTRAAELFKNAAIASGLRGKVKSNFRLKELKNMKSGLPTTKSDNFPIPLVKQKGGQYTGFEISSHNDDFIIKIPFGRWQVRKEVDKYRPWEKFNFEQVRKSPKPICLLLSTQRRKRNKGWSKDEGTEAEIRKVMNGDYQTSYIEVKRGSKIGEKSAWMLSLSIDVPKIDKGVDPSIIGGIDVGVKSPLVCAINNAFNRYSISDNNLFHFNKKMFARRRILLKKNRHKRAGHGVKNKLKSISILTEKSKRFRKKLIERWACEIADFFIKNKVGTVQMENLESMKRKEDSYFNIRLRGFWPYAEMQNKIEFKLKQYGIEIRKVAPNNTSKTCSKCGHLNNHFNFEYRKKNKFPHFKCEKCNFKEDADYNAALNISNPKLKSTKGEP

SEQ ID NO: 1481 - protein, 726 aa, synthetic construct
SEVGFSHEYWMRHALSLAKRARDEREVPVGAVLVLNNRVIGVGWNRAISLQDPTAHAEIMALRQGGLVMQNYRLSDATLYVTFEPCVMCAGAMIHSRIGRVVFGVRNSKRGAAGSLMNVLNYPGMNHCVEITEGILVDECAALLCDFYRMPRQVLSAQKKAQSSVSSGGSSGGSNDSETPGASGSVTPKSSVGGSAGSTKNTITKTLKLRIVRPYNSAEVEKIVADEKNNREKIALEKNRDKVKEACSKHLKVAAYCTTQVERNACLFCKARKLDDKFYQKLRGQFPDAVFWQEIGEIFRQLQKQAAEIYNQSLIELYYEIFIKGRGFANASSVEHYLSDVCYTRAAELFKNAAIASGLRGKVKSNFRLKELKNMRSGLPTTKSDNFPIPLVKQKGGQYAGFEISSHNDDFIIKIPFGRWQVKKEIDRYRPWEKFDFEQVRKSPKPISLLLSTQRRKRNKGWSKDEGTAAEIRRVMNGDYQTSYIEVKRGSKIGEKSAWMLSLSIDVPKIDKGVDPSIIGGIDVGVKSPLVCAINNASSRYSISDNDLFRFNKKMFARRRILLKKNRHKRAGHGAKNKLKPISILTGKSERFRKKLIERWACEIADFFVKNKVGTVQMENLESMKRKEDSYFNIRLRGFWPYAEMQNKIEFKLKQYGIEVRKVAPNNTSKTCSKCGHLNNYFDFEYRKKNKFPHFKCEKCNFKENADYNAALNISNPKLRSTKEEP

SEQ ID NO: 1482 - protein, 726 aa, synthetic construct
SEVEFSHEYWMRHALTLAKRARDEREVPVGAVLVLNNRVIGEGWNRAIGLHDPTAHAEIMALRQGGLVMQNYRLIDATLYVTFEPCVMCAGAMIHSRIGRVVFGVRNSKHGAAGSLVNVLNYPGMNHRVEITEGILADECAALLCDFYRMPRQVFNARKKAQSSINPSGSSGGSSGSVTPGTSESATPESSGGGFGGSAKNTITKTLQLRIVRPYNSAEVEKIVADEKNNREKIALEKNKDKVKEACSKHLKVASYCTTQVERNACLFCKARKLDDKFYQKLRGQFPDAVFWQELGEIFRQLQKQAAEIYNQSLIELYYVIFIKGKGLANASSVEHYLSDVCYTRAAELFKNAAIASGLRGKVKSNFKLKELKSMKSGLPSTKSDNFPIPLVKQRGGQYTGFEISSHNDDFIIKIPFGRWQAKKEIDKYRPWEKFDFEQVRKSPKPISLLLSTQRRKRNRGWSKDEGTEAEIRKVMNGDYQTSYIEVKRGSKIGEKSAWMLNLSIDVPKIDKGVDPSIIGGIDVGVKSPLVCAINNAFSRYSISDNDLFRFNKKMFARRRILLGKNRHKRAGHGVKNKLKPITILTEKSGRFRKKLIERWACEIADFFVKNKVGTVQMENLESMKRKEDSYFNIRLRGFWPYAEMQNKIEFKLKQYGIKVRKVAPNNTSKTCSKCGHLNNYFSFEYRKKNKFPHFKCEKCNFKENADYNAALNISNPKLKGTKEEP

SEQ ID NO: 1483 - protein, 726 aa, synthetic construct
SEVEFSHEYWMRHALTLAKRARDEREVPVGAVLVLNNRVIGEGWNRTTGLHDPTAHAEIMALRQGGLVMQNHRLVDATLYVTFEPCVMCAGAMIHSRIGRVVFGVRNSKRGAAGSLMNVLNYPGMNHCVEITEGILVDECAALLCDFYRMPRQVLNAQKKAQSSISPGGSSGGSSGSEAPGASESVTPKSSGGSSGGSAKNTITKTLKLRIVRPYNSAEVEKIVADEKNNREKIALEKNKGKVKEACSKHLEVAAYCTTQVERNACLFCKARKLDDKFYQKLRGQFPDAVFWQELGEIFRQLQKQAAEIYNQSLIELYYEIFIKGKGFANASSVEHYLSDVCYTRAAELFKNAAVASGLRGKVKSNFRLKELKNTKSGLPTTKSDNFPIPLVKQKGGQYTGFEISSHNDDFIIKIPFGRWQVKEEIDKYRPWEKFDFEQVRKNPKPISLLLSTQRRKRNKGWSKDEGTEAEIRRVMNGDYQTSYIEVKRGSKIGEKSTWMLNLSIDVPKIDKGVDPSIIGGIDVGVKSPLVCAINNAFSRYSISDNDLFRFNKKVFARRRILLKKNRHKRAGHGTKNKLKPITILTEKSGRFRKKLIERWACEIANFFIKNKVGTVQMENLESMKRKEDSYFNIRLRGFWPYAEMQNKIEFKLKQYGIKIRRVAPNNTSKTCSKCGHLNNYFSFEYRKKNKFPHFKCEKCNFKEDADYNAALNISNPKLKSTKEEP

SEQ ID NO: 1484 - protein, 726 aa, synthetic construct
SEVEFSHEYWMRHALTLAKRARDEREVPVGAVLVLNNRVIGEGWNRAIGLHDPTAHAEIMALRQGGLVTQNYRLIDATLYVTFEPCVMCAGAMVHSRIGRVVFGVRNSKRGAAGSLMNVLDHPGMDHRVEITEGILADECAALLCDFYRMPRQVFNAQKKAQSSINSGGPSGGSSGSETPGASESVTPKSSGGSSAGSTKNTITKTLKLRIVRPYNSAEVEKIVADEKNNRERIALEKNKDKVKEACSKHLKVAAYCTTQVERNACLFCKARKLDDKFYQKLRGQFPDAVFWQETGEIFRQLQRQAAEIYNQSLIELYYEIFIKGKGFANASSVEHYLSDVCYTRAAELFKNAAIASGLRGKVKGNFRLKELKNMKSGLPTTKSDNFPIPLVRQKGGQYTGFEISSHNDDFIIKIPFGRWQVKKEIDKYRPWEKFDFEQVRKSPKPISLLLSTQRRKRNKGWSKDEGTEAEIRKVMNGDYQTSYIEVKRGSKTGEKSAWMLNLSIDVPKIDKGVDPSIIGGIDVGVKSPLVCAINNAFSRYSISDNDLFRFNKKMFARRRILLKKNRHKRAGHGAKNKLKPISVLTGKSERFRKKLIERWACEIADFFIKNKVGTVQMENLESMKRKEDSYFNIRLRGFWPYAEMQNKIEFKLKQYGIEIRKVAPNNTSKTCSKCGHLNNYFNFEYRKKNKFPHFKCEKCNFKENADYNAALNISNPKLKSTKKEP

SEQ ID NO: 1485 - protein, 726 aa, synthetic construct
SEVEFSHEYWMRHALTLAKRARDEREVPVGAVLVLNNRVIGEGWNRAIGLHDPTAHAEVMALRQGGLVMQNYRLTDATLYVTFEPCVMCAGAMIHSRIGRVVFGVRNSKRGAAGSLVNVLNYPGMNHCVEITEGILVDECAALLCDFYRMPRQVLNAQKKAQSSTNPGGSSGGSSGSETPGTSESATPESPGGSSGGSAKNTITKTLKLRIVRPYNSAEVEKIVADEKNNREKIALEKNKDKVKEACSKHLKVASYCTTQVERNACLFCKARKLDDKFYQKLRGQFPDAVFWQELGEIFRQLQKQAAEIYNQSLIELYYEIFIKGKGFANASSVEHYLSDVCYTRAAELFKNAAIASGLRGKVKSNFRLKELKNMKSGLPTTKSDNFPIPLVKQKGGQYTGFEISSHNDDFVIKIPFGRWQVKKEIDKYRPWEKFDFEQVRKSPKPISLLLSTQRRKRNKGWSKDEGTEAEIRKVMNGDYQTSYIEVKRGSKIGEKSAWMLNLSIDVPKIDKGVDPSIIGGIDVGVKSPLVCAINNAFSRYSISDNDLFRFNKKMFARRRILLKKSKHKRAGHGAKNKLKPITILTEKSGRFRKKLIERWACEIADFFIKNKVGTVQMESLESMKRKEDSYFNIRLRGFWPYAEMQNKIEFKLKQYGIEIRKVAPNNTSKTCSKCGHLNNYFNFEYRKKNKFPHFKCERCNFKENADYNAALNISNPKLKSTKEEP

SEQ ID NO: 1486 - protein, 726 aa, synthetic construct
SEVEFSHEYWMRHALTLAKRARDEREVPVGAVLVLNNRVIGEGRNRAIGLHDPTAHAEIMALRQGGLVMQNYRLIDATLYVTFEPCVMCAGAMIHSRIGRVVFGVRNSRRGAAGSLINVLNYPGMNHRVEITEGILADECAALLCDFYRMPRQVLNAQRKAQSSSNSGGSSGCSSGSETPGASESVTPKSSGGSSGGSAKNTITKTLKLRIVRPYNSAEVEKIVADEKNNREKIALEKNKGKVKEACSKHLEVAAYCTTQVERNACLFCKARKLDDKFYQRLRGQFPDAVFWQELGEIFRQLQRQAAEIYNQSLIELYYEIFIKGKGFATASSVEHYLSDVCYTRAAELFKNAAIASGLRGKVKSNFRLKELKNMRSGLPTTKSDNFPIPLVKQKGGQYTGFEISSHNDDFIIKIPFGRWQVKKEIDKYRPWEKFDFEQVRKSPKPISLLLSTQRRKRNKGWSKDEGTEAEIRKVMNGDYQTSYIEVKRGSKIGEKSAWMLNLSIGVPKIDKGVDPSIIGGIDVGVKSPLVCAINNAFSRYSISDNDLFHFNKKMFARRRILLKKNRHKRAGHGAKNKLKPISILTEKSKRFRKKLIERWACEIADFFIKNKVGTVQMENLESMKRKEDSYFNIRLRGFWPYAEMQNRIEFKLKQYGIEIRKVAPNNTSKTCSKCGHLNNYFNFEYRKKNKFPHFKCEKCNFKENADYNAALNISNPKLKSTKEES

SEQ ID NO: 1487 - protein, 726 aa, synthetic construct
SEVEFSHEYWMRHALTLAERARDEHEVPVGAVLVLNNRVIGEGWNRAIGLHDPTAHAEIMALRQGGLVMQNYRLIDATLYVTFEPCVMCAGAMIHSRIGRVVFGVRNSKRGAAGSLTNVLNYPGMNHRVEITEGILVGECAALLCDFYRMPRQVFNAQKKAQSTINTGGSSGGSSGSETPGTSESPTPESSGSSPGGSAKNTITKTLKLRIVRPYNSAEVEKIVADEKNNREKIALEKNKDKVKEACSKHLKVAAYCTTQVERSACLFCKARKLDDKFYQKLRGQFPDAVFWQELGGIFRQLQKQAAEIYNQSLIELYYEIFIKGKGITNASRVEHYLSDVCYTRAAELFKNAAIASGLRGKVKSNLRLKELKNMKSGLPTTKSDNFPIPLVKQKGGQYTGFEISSHNDDFIIKIPFGRWQAKKEIDRYRPWEKFDFEQVRKSPKPISLLLSTRRRKRNKGWSKDEGTEAEIRKVMNGDYQTSYIEVKRGRKIGEKSVWMLNLSIDVPKIDKGVDPSTIGGIDVGVKSPLVCAINNAFSRYSISDNDLFRFNKKMFARRRILLKKNRHRRAGHGAKNKLKPIAVLAKKSEGFRKKLIERWACEVADFFIKNKVGTVQMENLESMKRREDSYFNIRLRGFWPYAEMQNKIEFKLKQYGIEVRKVAPNNTSKTCSKCGHLNNYFNFEYRKRNKFPHFKCEKCNFKENADYNAALNISNPKLKGTKEEP

SEQ ID NO: 1488 - protein, 726 aa, synthetic construct
SEVEFSHEYWMRHALTLAKRARDEREVPVGAVLVLNNRIIGEGWNRAIGLHDPTAHAEIMALRQGGLVMQNYRLIGATLYVTFEPCVMCAGAMVHSRIGRVVFGVRNSKRGAAGSLMNVLDYPGMGHRVEITEGILADECAALLCDFYCVPRQVFNAQKRAQSSINSGGSSGGSSGGETPGTSESATPESSGGGSSGSAKNTITKTLQLRIVRPYNSAEVEKIVADEKNNREKIALEKNKDKVKEACSEHLKVAAYCTTQVERNACLFCKARKLDDGFYQKLRGQFPDAVFWQEIGEIFRQLQKQAAEIYNQSLIELYYEIFIKGKGFANASSVEHYLSDVCYTRAAELFKNAAIASGLRGKVKSNFRLKELKNMKSGLPTTKSDNFPIPLVKQKGGQYTGFEISSHNDDLIVKIPFGRWQVKKEIDRYRPWEKFDFEQVRKSPKPISLLLSTQRRKRNKGWSKDEGTEAEIRKVMNGDYQTSYIEVRRGSKIGEKNAWMLSLSIDVPKIDKGVDPSIIGGIDVGVKSPLVCAINNAFSRYSISDNDLFRFNKKMFARRRILLKKNRHKRAGHGAKNKLKPISILTGKSERFRKKLIERWACEIADFFIKNKVGTVQMENLESMKRKEDSYFNIRLRGFWPYAEMQNKIEFKLKQYGIEIRKVAPNNTSRTCSKCGHLNNYFNFEYRKKNKFPHFRCEKCNFKEDADYNAALNISNPKLKSTKEEP

SEQ ID NO: 1489 - protein, 726 aa, synthetic construct
SEVEFSHEYWMRHALTLAKRARDEREVPVGAVLVLNNRVIGVGWNRAVGLHDPTAHAEIMALRQGGLVMQNYRLIEATLYVTFEPCIMCAGAMIHSRIGRVVFGVRNSKRGAAGSLMNVLNYPGMNHRVEITEGILADECAALLCDYYRMPRQVFNARKKAQSSINSGGSSDGGSGSETPGTSESATPESSGGSSGGSAKNTITKTLKLRIVRPYNSAEVEKIVADEKSNREKIALEKNKDKVKEACSEHLKVAAYCTTQVERSACPFCKARKLDDKFYQKLRGQFPDAVFWQEIGEIFRQLQRQAAEIYNQSLIELYYEIFIKGKGFANASSVEHYLSDVCYTRAAELFKNAAIASGLRGKVKSNFRLKELKNMRSGLPTAKSDNFPIPLVKQKGGQYTGFEISSHNDDFIIKIPFGRWQVKKEIDKYRPWEKFDFEQVRKSPKPISLLLSTQRRKRNKGWSKDEGTEAEIRKVMNGDYQTSYIEVKRGSKIGEKSAWVLNLSIDVPKIDKGVDPSIIGGIDVGVKSPLVCAINNSFSRYSICDNDLFRFNKKMFARRRILLKKNRHKRAGHGAKNKLKPISILTEKSKRFRKKLIERWACEIADFFIKNKVGTVQMENLESMKRKEDSYFNIRLRGFWPYAEMQNKIEFKLKQYGIEIRKVAPNNTSKTCSKCGHLNNYFNFEYRRKNKFPHFKCEKCNFKEDADYNAALNISNPKLKSTKEEP

SEQ ID NO: 1490 - protein, 726 aa, synthetic construct
SEVEFSHEYWMRHALTLAKRARDEREVPVGAILVLNNRVIGEGWNRAIGLHDPTAHAEIMALRQGGLVMQNYRLINATLYVTFEPCVMCAGAMIHSRIGRVVFGVRNSKHGAAGSLVNVLNYPGMNHRVEITEGILADECAALLCDFYRMPRQVFNARKKAQSSINSGGSSGGGSGGETPGTSESATQESSGGSSGGSAKNTITKTLKLRIVRPYNSAEVEKIVADEKNNREKIALEKNKDKVKEACSKHLKVAAYCTTQVERNACLFCKARRLDDKFYQKLRGQFPDAVFWQEIGEIFRQLQKQAAEIYNRSLIELYYEIFIKGKGIANASRVEHYLSDVCYTRAAELFKNAAIASGLRNRIKSNFRLKELKNMKSGLPTTKSDNFPIPLVKQKGGQYTGFEISSHNDDFIIKIPFGRWQVKKEIDKYRPWEKFDFEQVRKSPKPISLLLSTQRRKRNKGWSKDEGTEAEIKKVMNGDYQISYIEVKRGSKIGEKSAWVLNLSVDVPKIDKGVDPSIIGGIDVGVKSPLVCAINNAFSRYSISDNDLFRFNKKVFARRRILLKKNRHKRAGHGTKNKLKPITILTEKSGRFRKKLIERWACEIANFFIKNKVGTVQMENLESMKRKEDSYFNIRLRGFWPYAEMQNKIEFKLKQYGIEIRKVAPNNTSKTCSKCGHLNNYFSFEYRKKNKFPHFKCEKCNFKEDADYNAALNISNPKLMSTKEGP

SEQ ID NO: 1491 - protein, 726 aa, synthetic construct
SEVEFSHEYWMRHALTLAKRARDEREVPVGAILVLNNRVIGEGWNRAIGLHDPTAHAEIMALRQGGLVMQNYRLTDATLYATFEPCVMCAGAMIHSRIGRVVFGVRNSKHGAAGSLMNVLNYPGMNHRVEITEGILADECAGLLCDFYRMPRQVFSARKKAQSSINPGGSSGGSSGGKAPGTSESATLESSGGSSGGSAKNSITKTLKLRIVRPYNSAEVEKIVADEKNNREKTALEKNKGKVKEACSKHLKVATYCTTQVERNACLFCKARKLDDKFYQKLRGQFPDAVFWQEIGEIFRQLQKQAAEIYNQSLIELYYEIFIEGKGSANARSVEHYLSDVCYTRAAELFKNAAIASGLRGKVKGNFRLKELKSMKSGLPTTKSDNFPIPLVKQKGGQYTGFEISSHNDDFIIKIPFGRWQVKKEIDKYRPWEKFDFEQVRKSPKPISLLLSTQRRKRNKGWSKDEGTEAEIRKVMNGDYQISYIEVKRGSKIGEKSAWMLSLSIDVPKIDKGVDPSIIGGIDVGVRSPLVCAIDNAFSRYSISDNDLFRFNKKMFARRRILLGKNRHKRAGHGVKNKLKPITILTEKSGRFRKKLIERWACEIADFFAKNKVGTVQMENLESMKRKEDSYFNIRLRGFWPYAEMQNKIEFKLKQYGIKVRKVAPNNTSKTCSRCGHLNNYFNFEYRKENKFPHFKCEKCNFKENADYNAALNISNPKLKSTKGEP

SEQ ID NO: 1492 - protein, 726 aa, synthetic construct
SEVEFSHEYWMRHALTLAKRARDEREVPVGAILVLNNRVIGEGWNRAIGLHDPTAHAEIMALRQGGLVMQNYRLIDATLYVTFEPCVMCAGAMIHSRVGRVVFGVRNSKHGAAGSLMNVLNYPGMNHRVEITEGILVDECAALLCDFYRMPRRVFNARKKAQSSIDPGGPSGGSSGSETPGTSESATPESSGGSSGGSAKNTITKTLKLRIVRPYNSTEVEKIVADEKNNREKIALEKNKDKVKEACSEHLKVAAYCTTQVERNACLFCKARKLDDRFYQKLRGQFPDAVFWQEIGEIFRQLQKQAAEIYNQSLIELYYEIFIKGKGFANASSVEHYLSDVCYTRAAELFKNAAIASGLRGKVKSNFRLKELKNMKSGLPTTKSDNFPIPLVKQKGGQYTGFEISSHNDDFIIKIPFGRWQVRKEIDKYRPWEKFNFEQVRKSPKPISLLLSTQRRKRNKGWSKDEGTEAEIRKVMNGDYQTSYIEVKRGSKIGEKSAWMLNLSIDVPKIDKGVDPSITGGIDVGVKSPLVCAINNALSRYSISDNDLFRFNKKMFARRRILLRKNRHKRAGHGARNKLKPITVLTEKSERFRKKLIERWACEIANFFIKNKVGTVQMENLESMKRKEDSYFNIRLRGFWPYAEMQNKIEFKLKQYGIKIRKVAPNNTSKTCSKCGHLNNYFSFEYRKKNKFPHFKCEKCNFKEDADYNAALNISNPKLKSTKEEP

SEQ ID NO: 1493 - protein, 726 aa, synthetic construct
SEVEFSHEYWMRHALTLAKRARDEREVPVGAILVLNNRVIGEGWNRAIGLHDPTAHAEIMALRQGGLVLQNYRLVDATLYVTFEPCVLCAGAMVHSRIGRVVFGARNSKRGAAGSLMNILNYPGMNHRVEITEGILADECAALLCDFYRMPRQVFNAQKKAQSTINSGGSSGGSSGSETPGTSESATPESSGGSSGGSAKNTITKTLKLRIVRPYNSAEVEKIVADEKDNRERIALEKNKGKVKEACSKHLRVAAYCTTQVERNACLFCKARKLDDKFYQELRGQFPDAVFWQEIGEIFRQLQKQAAEIYNQSLIELYYEIFIKGKGIVNASSVGHYLSDVCYTRAAELFKNAAIASGLRSKIKSNFRLKELRNMRGGLPTTKSDNFPIPLVKQKGGQYTGFEISNHNGDFIIKIPFGRWQVKKEISKHRPWEKFDFEQVRKSPKPISLLLSTQRRKRNKGWGKDEGTEAEIRKVMNGDYQTSYIEVKRGSKIGEKSAWMLNLSIDVPKIDKGVDPSIIGGIDVGVKSPLVCAINNALSRYSISDNDLFHFNKKMFARRRILLRKNRHKRAGHGAKNKLKPISILTEKSKRFRKKLIERWACEIADFFIKNKVGTVQMENLESMKRKEDSYFNIRLRGFWPYAEMQNKIEFKLKQYGIEIRKVAPNNTSKTCSKCGHLNNYFSFEYRKKNKFPHFKCEKCNFKENADYNAALNISNPKLKSTKEEP

SEQ ID NO: 1494 - protein, 726 aa, synthetic construct
SEVEFSHEYWMRHALTLAKRARDEREVPVGAILVLNNRVIGEGWNRTTGLHDPTAHAEIMALRQGGLVMQNHRLVDATLYVTFEPCVMCAGAMIHSRIGRVVFGVRNSKRGAAGSLTNVLNYPGMNHRVEITEGILVDECAALLCDFYRMPRQVFNAQKKAQSTINSGGSSGGSSGSETPGTSESPTPESSGGSPGGSAKNTITKTLKLRIVRPYNSAEVEKIVADEKNNREKIALEKNKDKVKEACSRHLKVAAYCTTQVERNACLFCKARKLDDKFYQKLRGQFPDAVFWQEIGEIFRQLQKQAAEIYNQSLIELYYEIFIKGKGFANASSVEHYLSDVCYARAAELFKNAAIASGLRGKVKSNFRLKELKNMKSGLPTTKSDNFPIPLVKQKGGQYTGFEISSHNDDFIIKIPFGRWQVKKEIDKYRPWEKFDFEQVRKSPKPISLLLSTQRRKRNRGWSKDEGTEAEIRKVMNGDYQTSYIEVKRGSKTGEKSAWMLNLSIDVPKIDKGVDPSIIGGIDVGVKSPLVCAINNAFSRYSISDNDLFRFNKKMFARRRILLKKNRHKRAGHGAKNKLKPISILTGKSERFRKKLIERWACEIADFFIKNKVGTVQMENLESMKRKEDSYFNIRLRGFWPYAEMQNKIEFKLKQYGIEIRKVAPNNTSKTCSKCGHLNNYFNFEYRKKNKFPHFKCEKCSFKENADYNAALNISNPKLKSTKEEP

SEQ ID NO: 1495 - protein, 726 aa, synthetic construct
SEVEFSHEYWMRHALTLAKRARDEREVPVGAILVLNNRVIGEGWNRAIGLHDPTAHAEIMALRQGGLVMQNYRLIDATLYVTFEPCVMCAGAMIHSRIGRVVFGVRNSKHGAAGSLVNVLNYPGMNHRVEITEGILADECAALLCDFYRMPRQVFNARKKAQSSINSGGSSGGSSGSETLGTSESATPESSGGSSGGSAKNTITKTLQLRIVRPYNSAEVEKIVADEKNNREKIALEKNKDKVKEACSKHLKVASYCTTQVERNACPFCKARKLDDKFYQKLRGQFPDAVFWQELGEILRQLQKQAAEIYNQSLIELYYEIFIKGKGFANASSVEHYLSDVCYTRAAELFKNAAIASGLRGKVKSNFRLKELKNMKSGLPTTKSDNFPIPLVKQKGGQYTGFEISSHNDDFIIKIPFGRWQVKEEIDKYRPWEKFDFEQVRKNPKPISLLLSTLRRKRNKGWSKDEGTEAEIRKVMNGDYQTSYIEVKRGSKIGEKSAWMLNLSIDVPKIDKGADPSIIGGIDVGVKSPLVCAINNAFSRYSISDNDLFRFNKKVFARRRILLKKNRHKRAGHGTKNKLKPITILTEKSGRFRKKLIERWACEIANFFIKNKVGTVQMENLESMKRREDSYFNIRLRGFWPYAEMQSKIEFKLKQYGIKIRKVAPNNTSKTCSKCGHLNNYFNFEFRKKNKFPHFKCEKCNFKEDADYNAALNISNPKLKSTKEEP

SEQ ID NO: 1496 - protein, 726 aa, synthetic construct
SEVEFSHEYWMRHALTLAKRARDEREVPVGAILVLNNRVIGVGWNRAIGLHDPTAHAEIMALRQGGLVTQNYRLIDATLYVTFEPCVMCAGAMIHSRIGRVVFGVRNSKHGAAGSLVNVLNYPGMNHRVEITEGILADECAALLCDFYRMPRQVFNARKKAQSSINSGGSSGDSSGSETPGTSESATPKSSGGSSTGSTKNTITKTLKLRIVRPYNSAEVEKIVADEKDNREKIALEKNKDKVKEACSKHLKVASYCTTQVERNACLFCKARKLDDKFYQKLRGQFPDAVFWQELGGIFRQLQKQAAEIYNQSLIELYYEIFIKGKGITNASRVEHYLSDVCYTRAAELFKNAAIASGLRSKVRSNFRLKELKNMKSGLPTTKSDNFPIPLVKQKGGQYTGFGISSHNSDFIIKIPFGRWQEKEEIDKYRPWEKFDFEQVRRSPKPISLLLSTQRRKKNKGWSKDEGTEAEIRRVMNGDYQTSYIEVKRGSKIGEKSAWMLNLSIDVPKIDKGVDPSIIGGIDVGVKSPLVCAINSAFSRYSISDNDLFHFNKKMFARRRILLKKNRRRRAGHGAKNKLKPITILTEKSARFRKKLIERWACEIADFFIKNKVGTVQMENLESMKRKEDSYFNIRLRGFWPYAEMQNKIEFKLKQYGIEIRRVAPNNTSRTCSKCGHLNNYFNFEYRRKYKFPHFKCEKCNFKEDADYNAALNISNPKLKSTKEEP

SEQ ID NO: 1497 - protein, 726 aa, synthetic construct
SEVEFSHEYWMRHALTLAKRARDEREVPVGAILVLNNRVIGEGWNRAIGLHDPTAHAEIMALRQGGLVMQNYRLSDATLYVTFEPCVMCAGAMIHSRIGRVVFGVRNSKRGAAGSLMNVLNYPGMNHRVEITEGILAGECAALLCDFYRMPRQVFNARKKAQSSISPGGSSGGSSGSETPGTSESATPESSGGSSGGSAKNTITKTLKLRIVRPYNSAEVEKIVADEKDSREKIALEKNKDKVKEACSKHLKVAAYCTTQVGRNACLFCKARKLDDKFYQKLRGQFPDAVFWQEISEIFRQLQKQAAEVYNQSLIELYYEIFIKGKGFANASSVEHYLSDVCYTRAAELFKNAAIASGLRGKVKSNFRLKELKNMKSGLPTTKSDNFPIPLVKQKGGQYTGFEISSHNDDFIIKIPFGRWQMKKEVDKYRPWEKFDFEQVRKSPKPISLLLSTQRRKRNKGWSKDEGTEAEIRKVMNGDYQTSYIEVKRGSKIGEKSAWMLNLSIDVPKIDKGVDPSIIGGIDVGVKSPLVCAINNAYSRYSISDNDLFHFNKKMFARRRILLKKTRHKRAGHGAKNKLKPVSILTEKSERFRKKLIERWACEIADFFIKNKVGTVQMENLESMKRREDSYFNIRLRGFWPYAKMQNKIEFKLKQYGIEIRKVAPNNTSKTCSKCGHLNNYFNFEYRKKNKFPHFKCEKCNFKESADYNAALNISNPKLKSTKEEP

SEQ ID NO: 1498 - protein, 726 aa, synthetic construct
SEVEFSHEYWMRHALSLAKRARDEREVPVGAVLVLNNRIIGEGWNRAIGLHDPTAHAEIMALRQGGLVMQNYRLTDATLYVTFEPCVMCAGAMIHSRIGRVVFGVRNSKHGAAGSLVNVLNYPGMNHRVEITEGILADECAALLCDFYRMPRQVFNARKKAQSSINSGGSSGGSSSSETPGTSESATSESSGGSSGGSARNTITKTLQLRIVRPYNSAEVEKIVADEKNRREKIALERNKDKVKEACSEHLKVAAYCTTQVERNACLFCKARKLDDRFYQKLRGQFPDAVFWQETGEIFRQLQRQAAEIYNQSLIELYYEIFIKGKGFANASSVEHYLSDVCYTRAAELFKNAAIASGLRGKVKSNFRLKELKNMKSGLPTTKSDNFPIPLVKQKGGQYTGFEISSHNDDFIIKIPFGRWQVKKEIDKYRPWEKFDFEQVRKSPKPISLLLSTRRRKRNKGWSKDEGTEAEIRKVMNGDYQTSYIEVKRGSKIGEKSAWMLNLSIDVPKIDKGVDPSIIGGIDVGVKSPLVCAINNAFSRYSISDNELFHFNKKMFARRRILLKKNGHKRAGHGAKNKLKPISALTEKSERFRKKLIERWACEIADFFIKNKVGTVQMENLESMKRKEDSYFNIRLRGFWPYAEMQSKIEFKLKQYGIEIRKVAPNNTSKTCSKCGHLNNYFSFEYRKKNKFPHFKCEKCNFKENADYNAALNISNPKLKSTKEEP

SEQ ID NO: 1499 - protein, 726 aa, synthetic construct
SEVEFSHEYWMRHALTLAKRARDEREVPVGAVLVLNNRVIGEGWNRAIGLHDPTAHAEIMALRQGGLVMQNYRLIDATLYVTFEPCVMCAGAMIHSRIGRVVFGVRNSKHGAAGSLMNVLNYPGMNHRVEITEGILADECAALLCDFYRMPRQVFSAQRKAQSSINPGGSSGGSSGSETPGTSESATPKSSGGGSAGSTKSTITKTLKLRIVRPYNSAEVEKIVADEKNSREKIALERNKDKVKEACSEHLKVAAYCTTQVERNACLFCKARKLDDKFYQKLRGQFPDAVFWQEIGEIFRQLQKQAAEIYNQSLIELYYEIFVKGKGFANASSVEHYLSDVCYTRAAELFKNAAIASGLRGKVKSNFRLKELKNMKSGLPTTKSDNFPIPLVKQKGGQYTGFEISSHNDDFIIKIPFGRWQARKEIDKYRPWEKFDFEQVRKSPKPISLLLSTQRRKRNKGWSKDEGTEAEIRKVMNGDYQTSYIEVKRGSKIGEKSAWMLNLSIDVPKIDKGVDPSIIGGIDVGVKSPLVCAINNAFSRYSISDNDLFHFNKKMFARRRILLKKNRHKRAGHGAKNKLKPISILTEKSKRFRKKLIERWACEIADFFIKNKVGTVQMENLESMKRKEDSYFNIRLRGFWPYAEMQNRIELKLKQYGIEIRRVAPNNTSRTCSKCGHLNNYFNFEYRKMNKFPHFKCEKCNFKENADYNAALNISNPKLKSAKEEP

SEQ ID NO: 1500 - protein, 726 aa, synthetic construct
SEVEFSHEYWMRHALTLAKRARDEREVPVGAVLVLNNRVIGEGWNRAIGLHDPTAHAEIMALRQGGLVMQNYRLTDATLYVTFEPCVMCAGAMIHSRIGRVVFGVRNSKRGAAGSLMNVLNYPGMDHRVEITEGILTDECAALLCDFYRMPRQVFNAQRKAQSNINPGSSSGGSSGSETPSTSESATPGSSGGSSGGSAKNTITKTLKLRIVRPYNSAEVEKIVADEKNNREKIALEKNKDKVKEACSEHLKVAAYCTTQVERNACPFCKARKLDDKFYRKLRGQFPDAVFWQEIGEIFRQLQKQAAEIYNQSLIELYYEIFIKGKGFANASSLEHYLSDVCYTRAAELFKNAAIASGLRNKVKSNFRLKELKSMKSGLPTTKSDNFPIPLVKQKGGQYTGFEISNHNSDFIIKIPFGRWQVKKEIDKYRPWEKFDFEQVRKSPKPISLLLSTRRRKRNKGWSKDEGTEAEIRKVMNGDYQTSYIEVKRGSKIGEKSAWMLNLSIDVPKIDKGVDPSIIGGIDVGVKSPLVCAINNAFGRYSISDNDLFHFNKKMFARRRILLKKNGHKRAGHGAKNKLKPITILTEKSKRFRKKLIERWACEIADFFIKNKVGTVQMENLESMKRREDSYFNIRLRGFWPYAEMQNKIEFKLKQYGIEIRKVAPNNTSKTCSKCGHLNNYFNFEYRKKNKFPHFKCEKCNFKENADYNAALNISNPKLMSTKEEP

SEQ ID NO: 1501 - protein, 726 aa, synthetic construct
SEVEFSHEYWMRRALTLAKRARDEREVPVGAVLVLNNRVIGVGWNRAVGLHDPTAHAEIMALRQGGLVMQNYRLIEATLYVTFEPCIMCAGAMIHSRIGRVVFGVRNSKRGAAGSLMNVLNYPGMNHRVEITEGILADECAALLCDFYRMPRQVFNAQRKAQSSINFGGSSGGSSGSGTPGTSESATPESSGGSSGGSAKNTITKTLKLRIVRPYNSAEVEKIVADEKNNREKIALEKNKDKVREACSEHLKVASYCTTQVERNACLFCKARKLDDKFYQKLRGQFPDAVFWQELGEIFRQLQKQAAEIYNQSLIELYYEIFIKGKGFANASSVEHYLSDVCYTRAAELFKNAAIASGLRGKVKSNFRLKELKNMKSGLPTTKSDNFPIPLVKQKGGQYTGFEISSHNDDFIIKIPFGRWQVKKEIDKYRPWEKFDFEQVRKSPKPISLLLSTQRRKRNKGWSKDEGTEAEIRKVMNGDYQTSYIEVKRGSKTGEKSTWMLNLSIDVPKIDKGVDPSIIGGIDVGVKSPLVCAINNSSSRYCICDNDLFRFNKKMFARRRILLKKNRHKRAGHGAKNKLKPITILTKKSERFRKKLIERWVCEVANFFIKNKVGTVQMENLESMKRKEDSYFNIRLRGLWPYAEMQNKIEFKLKQYGIEVRKVAPNNTSKTCSKCGHLNNYFNFEYRKRNKFPHFKCEKCNFKENADYNAALNISNPKLKGTKEEP

SEQ ID NO: 1502 - protein, 726 aa, synthetic construct
SEVEFSHEYWMRHALTLAKRARDEREVPVGAVLVLNNRIIGEGWNRAIGLHDPTAHAEIMALRQGGLVLQNYRLIDATLYVTFEPCVMCAGAMVHSRIGRVVFGVRNSKRGAAGSLMNVLDYPGMGHRVEITEGVLADECAALLCDFYCMPRQVFNAQKRAQSSINSGGSSGGSSGSETPGTSESATPESSGGGSSGSAKNTITKTLQLRIVRPYNSAEVEKVVADEKNNREKIALEKNKDKVKEACSKHLKVASYCTTQVERNACPFCKARKLDDKFYQKLRGQFPDAVFWQELGEILRQLQKQAAEIYNQSLIELYYEIFIKGRGFANASSVEHYLSDVCYTRAAELFKNAAIASGLRGKVKSNFRLKELKNMKSGLPTTKSDNFPIPLVKQKGGQYTGFEISSHDDDFIIKVPFGRWQVKKEIDKYRPWEKFDFEQVRKSPKPISLLLSTQRRKRNKGWSKDEGTEAEIRKVMNGDYQTSYIEVKRGSKTGEKSAWMLNLSIDVPKIDKGVDPSIIGGIDVGVKSPLVCAINNAFSRYSISDNDLFRFNKKMFARRRILLKKNKHKRAGHGAKNKLKPISILTGKSERFRKKLIERWACEIADFFIKNKVGTVQMENLESMKRKEDSYFNIRLRGFWPYAEMQSKIEFKLKQYGIEIRKVAPNNTSKTCSKCGHLNNYFNFEYRKKNKFPHFKCEKCNFKENADYNAALNISNPKLKSTKEEP

SEQ ID NO: 1503 - protein, 726 aa, synthetic construct
SGVEFSHEYWMRHALTLAKRARDEREVPVGAVLVLNNRVIGEGWNRAIGLHDPAAHAEIMALRQGGLVMQNYRLIGATLYVTFEPCVMCAGAMIHSRVGRVVFGVRNNKHGAAGSLVNVLNYPGMNHRVEITEGILADECAALLCDFYRMPRQVFNARKKAQSSINPGSSSGGSGGSETPGTSESATPESSGGSSGSSAKNTITKTLKLRIVRPYNSAEVEKIVADEKNNREKIALEKNKDKVKEACSKHLKVASYCTTQVERNACPFCKARKLDDKFYQKLRGQFPDAVFWQEIGEIFRQLQKQAAEIYNQSLIELYYEIFIKGKGFANASSVEHYLSDVCYSRAAELFKNAAIASGLRGKVKSNFRLKELKNMKSGLPTTKSDNFPIPLVKQKGGQYTGFEISSHNDDFIIKIPFGRWQVKKEIDKYRPWEKFDFEQVRKSPKPISLLLSTQRRKRNKGWSKDEGTEAEIKKVMNGDYQISYIEVKRGSKIGEKSAWMLNLSVDVPKIDKGVDPSIIGGIDVGVKSPLVCAINNALSRYSISDNDLFHFNKRMFARRRILLRGNRHKRAGHGAKNKLKPISILTEKSKRFRKKLIERWACEIADFFIKNEVGTVQMENLESMKRREDSYFNIRLRGFWPYAEMQSKIEFKLKQYGIVVRKVAPNNTSKTCSKCGHLNNYFNFEFRKKNKFPHFKCEKCNFREDADYNAALNISNPKLKSTKGEP

SEQ ID NO: 1504 - protein, 726 aa, synthetic construct
SGVEFSHEYWMRHALTLAKRARDEREVPVGAILVLNNRVIGEGWNRAIGLHDPTAHAEIMALRQGGLVMQNYRLIDATLYVTFEPCVMCAGAMIHSRIGRVVFGVRNNKHGAAGSLVNVLNYPGMNHRVEITEGILADECAALLCDFYRMPRQVFNARKKAQSSINSGGSSGGSSGSETPGTCESATPGSSGGGSGGSARGTITKTLKLRIVRPYNSAEVEKIVADEKNNREKIALEKNKDKVKEACSKHLKVAAYCTTQVERNVCLFCKARKLDDKFYQKLRGQFPDAVFWQEIGEIFRQLQKQAAEIYNQGLIELYYEIFIKGKGIANASSVGHYLSDVCYTRAAELFKNAAIASGLRSKIKSNFRLKELKSMKSGLPTTKSDNFPIPLVKQKGGQYAGFEISNHNGDFIIKIPFGRWQVKKEVDRYRPWEKFDFEQVRKSPKPISLLLSTQRRRRNKGWSKDEGTEAEIRKVMNGDYQTSYIEVKRGSKIGEKSAWMLNLSIDVPKIDKGVDPSIIGGIDVGVKSPLVCAINNAFSRYSISDNDLFHFNKKMFARRRILLKKNRHKRAGHGAKNKLKPISILTEKSKRFRKKLIERWACEIADFFIKNKVGTVQMENLESMKRKEDSYFNIRLRGFWPYAEMQNKIEFKLKQYGIEIRKVAPNNTSKTCSKCGHLNNYFNFEYRKMNKFPHFKCEKCNFKENADYNAALNISNPKLKSTKEEP

SEQ ID NO: 1505 - protein, 726 aa, synthetic construct
SEVEFSHEYWMRRALTLAKRARDEREVPVGAVLVLNDRVIGEGWNRAVGLHDPTAHAEIMALRQGGLVMQNHRLIEATLYVTFEPCIMCAGAMIHSRIGRVVFGVRNSKRGAAGSLMNVLNYPGMNHRVEITEGILADECAALLCDYYRMPRQVFNARKKAQSSINPGGSSGGSGGSETPGTSESATPENSGGSSGSSAKNTITKTLKLRIVRPYNSAEVEKIVADEKNNREKIALEKNKDKVKEACSRHLKVAAYCTTQVERNACLFCKARRLDDKFYQKLRGQFPDAVFWQEIGEIFRQLQKQAAEIYNQSLVELYYEILIKGKGIANASSVEHYLSDVCYTRAAELFKNAAIASGLRNKVKSNFRLKELRNMKSGLPTTMSDNFPIPLVKQKGGQYTGFEISSHDDDFIIKIPFGRWQVKKEFDKYRPWEKFDFEQVRKSPKPISLLLSTQRRKRNKGWSKDEGTEAEIRKVMNGDYQISYIEVKRGSKIGEKSAWMLSLSIDVPKIDKGVDPSIIGGIDVGVKSPLVCAINNAFSRFSISDNDLFHFNKKMFARRRILLKKNRHRRAGHGVKNKLKPITILAEKSKRFRKKLIERWACEIADFFVKNKVGTVQMENLESMKRKEDSYFNIRLRGFWPYAEMQNKIEFKLKQYGIEIRKVAPNNTSRTCSKCGHLNNYFNFEYRKKNKFPHFKCEKCDFKENADYNAALNISNPKLKSTKEEP

SEQ ID NO: 1506 - protein, 726 aa, synthetic construct
SEVEFSHEYWMRHALTLAKRARDEREVPVGAVLVLNNRVIGEGWNRAIGLHDPTAHAEIMALRQGGLAMQNYRLVDATLYVTFEPCVLCAGAMVHSRIGRVVFGVRNSKRGAAGSLMNVLNHPGMNHRVEITGGILADECAALLCDFYRMPRQVFNAQKKARSNINSGGSSGGSSGSETLGTSESATPESSGGSSGGSAKNTITKTLKLRIVRPYNSPEVEKIVADEKNNREKIALEKNKDKVKEACSEHLKVATYCTTQVERNACLFCKARKLDDKFYQKLRGQFPDAVFWQEIGEIFRQLQKQAAEIYNQSLIELYYEIFIEGKGSANARSVEHYLSDVCYTRAAELFKNAAIASGLRGKVKSNFRLKELKNMRSGLPTTKSDNFPIPLVKQKGGQYTGFEISSHNDDFIIKIPFGRWQVKKEIDKYRPWEKFDFEQVRKSPKPISLLLSTQRRKRNKGWSKDEGTEAEIRKVMNGDYQTSYIEVKRGSKIGEKSAWMLNLSIGVPKIDKGVNPSIIGGIDVGVKSPLVCAINNAFSRYSISDNDLFHFNKKMFARRRILLKKNRHKRAGHGAKNKLKPISILTEKSKRFRKKLIERWACEIADFFIKNEVGTVQMENLESMKRKEDSYFNIRLRGFWPYAEMQNRIEFKLKQYGIEVRKVAPNNTSKTCSKCGHLNNYFNFEYRKKNKFPYFKCEKCNFKENADYNAALNISNPKLKSTKEEP

SEQ ID NO: 1507 - protein, 725 aa, synthetic construct
SEVEFSHEYWMRHALTLAKRARDEREVPVGAVLVLNNRVIGEGWNRAIGLHDPTAHAEIMALRQGGLVMQNYRLIGATLYVTFEPCVMCAGAMIHSRIGRVVFGVRNSKHGAAGSLVNVLNYPGMNHRVEITEGILADECAALLCDYYRMPRQVFNAQKKAQSTINSGGSSGGSSGSETPGTSESPTPESSGGSPGGSAKNTITKTLKLRIVRPYNSAEVEKIVADEKNNREKIALEKNKDKVKEACSKHLKVAAYCTTQVERNACLFCKARKLDDKFYQKLRGQFPDAVFWQEIGEIFRQLQKQAAEIYNQSLIELYYEIFIKGKGFANASSVEHYLSDVCYTRAAELFKNAAIASGLRGKVKSNFRLKELKNMRSGLPTTKSDNFPIPLVKQKGGQYAGFEISSHNDDFIIKIPFGRWQAKEEIDKYRPWEKFDFEQVRKSPKPISLLLSTRRRKRNKGWSKDEGTEAEIRKVMNGDYQTSYIEVKRGSKIGEKSAWMLNLSIDVPKIDKGVDPSIIGGIDVGVKSPLVCAINNAFGRYSISDNDLFHFNKKMFARRRILLKKNRHKRAGHGAKNKLKPITILTEKSKRFRKKLIERWACEIADFFIKNKVGTVQMENLESMKRKEDSYFNIRLRGFWPYAEMNKIEFKLKQYGIKVRKVAPNNTSKTCSKCGHLNNYFSFEYRKKNKFPHFKCEKCNFKENADYNAALNISNPKLKSTKEES

SEQ ID NO: 1508 - protein, 726 aa, synthetic construct
SEVEFSHEYWMRHALTLAKRARDEREVPVGAVLVLNNRVIGEGWNRAIGLHDPTAHAEIMALRQGGLVMQSYRLADATLYVTFEPCVMCAGAMIHSRIGRVVFGVRNSKHGAAGSLMNVLNYPGMNHRVEITEGILADECAALLCDFYRMPRRVFNAQKKAQSSINSGGSSGGCSGSEMPGASESVTPKSSGGSSAGSTKNTITKTLKLRIVRPYNSAEVEKIVADEKNSREKIALERNKDKVKEACSEHLKVAAYCTTQVERNACLFCKARKLDDRFYQKLRGQFPDAVFWQETGEIFRQLQRQAAEIYNQSLIELYYEIFIKGKGFANASSVEHYLSDVCYTRAAELFKNAAIASGLRGKVKSNFRLKELKNMKSGLPTTKSDNFPIPLVKQKGGQYTGFEISSHNDDFIIKIPFGRWQVKKEIDKYRPWEKFDFEQVRKSPKPISLLLSTQRRKRNKGWSKDEGTEAEIRKVMNGDYQTSYIEVKRGSKTGEKSTWMLNLSIDVPKIDKGVDPSIIGGIDVGVKSPLVCAINNALSRYSISDNDLFHFNKKMFARRRILLRKNRHKRAGHGARNKLKPITVLTEKSERFRKKLIERWACEIANFFIKNKVGTVQMENLESMKRREDSYFNTRLRGFWPYAEMQNKIEFKLKQYGIKIRKVAPNNTSKTCSKCGHLNNYFNFEFRKKNKFPHFKCEKCNFKEDADYNAALNISNPKLKSTKEEP

SEQ ID NO: 1509 - protein, 726 aa, synthetic construct
SEVEFSHEYWMRHALTLAKRARDEREVPVGAVLVLNNRVIGEGWNRAIGLHDPTAHAEIMALRQGGLVMQNYRLVDATLYVTFEPCVLCAGAMVHSRIGRVVFGVRNNKRGAAGSLMNVLNYPGMNHRVEITEGILADECAALLCDFYRMPRQVFNARRKARSNINSGGSSGGSGDSETPGTSESATPESSGGSSAGSTKNTITKTLKLRIVRPYNSAEVEKIVADEKNNREKIALEKNKDKVKEACSKHLKVAAYCTTQVERNACQFCKARKLDDKFYQKLRGRFPDAVFWQELGEILRQLQKQAAEIYNQSLIELYYEIFIKGRGFANASSVEHYLSDVCYTRAAELFKNAAIASGLRGKVKSNFRLKELKNMKSGLPTTKSDNFPIPLVKQKGGQYTGFEISSHNDDFIIKIPFGRWQVKKEINKYRPWEKFDFEQVRKSPKPISLLLSTQRRKRNKGWSKDEGTEAEIRKVMNGDYQTSYIEVKRGSTIGEKSVWMLNLSINVPKIDKGVDPSIIGGIDVGVKSPLVCAINNAFSRYSISDNDLFRFNKKMFARRRILLKKSKHKRAGHGAKNKLKPITILTEKSGRFRKKLIERWACEIADFFIKNKVGTVQMENLESMKRKEDSYFNIRLRGFWPYAEMQNKIEFKLKQYGIEIRKVAPNNTSKTCSKCGHLNNYFNFEYRKKNKFPHFKCEKCSFKENADYNAALNISNPKLKSTKEES

SEQ ID NO: 1510 - protein, 726 aa, synthetic construct
SEVEFSHEYWMRHALTLAKRARDEREVPVGAILVLNNRVIGVGWNRAIGLHDPTAHAEIMALRQGGLVMQNYRLIDATLYVTFEPCVMCAGAMIHSRIGRVVFGVRNSKHGAAGSLVNVLNYPGMNHRVEITEGILADECAALLCDFYRMPRQVFGARRKAQSSINPSGSSGGSSGSETPGTSESPTPESPGGSYGGSAKNTITKTLKLRIVRPYNSAEVEKIVADEKNNREKIALEKNKDKVKEACSKHLKMASYCTIQVERNACPFCKARKLDDKFYQKLKGQFPDAVFWQEIGEVFRQLQKQAAEIYNQSLIELYYEIFIKGKGFANASSVEHYLSDVCYTRAAELFKNAAIASGLRGKVKSNFRLKELKNMKSGLPTTKSDNFPIPLVKQKGGQYTGFEISSHNDDFIIKIPFGRWQVKKEIDRYRPWEKFDFEQVRKSPKPISLLLSTQRRKRNKGWSKDEGTEAEIRKVMNGDYQTSYIEVKRGSKIGEKSAWMLNLSIDVPKIDKGVDPSIIGGIDVGVKSPLVCAINNAFSRYSISDNDLFHFNKKVFARRRILLKKNRHRRAGHGAKNKLKPITILTEKSKRFRKKLIERWACEIADFFIKNKVGTVQMENLESMKRKEDSYFNIRLRGFWPYAEMQNKIEFKLKQYGIEIRKVAPNNTSKTCSKCGHLNDYFNFEYRKKNKFPHFKCEKCNFKENADYNAALNISNPKLKSTKEEP

SEQ ID NO: 1511 - protein, 726 aa, synthetic construct
SEVEFSHEYWMRHALTLAKRARDEREVPVGAILVLNNRIIGEGWNRAIGLHDPTAHAEIMALRQGGLVMQNYRLIDATLYVTFEPCVMCAGAMIHSRIGRVVFGVRNSKHGAAGSLVNVLNYPGMNHRVEITEGILADECAALLCDFYRMPRQVFNARKKAQSSINPGGSSGGSGGSETPGTSESATPESSGGSSGGSAKNTITKTLKLRIVRPYNSAEVEKIVADEKDNREKIALEKNKDKVKEACSKHLKVAAYCTTLVERNACLFCKARKLDDKFYQKLRGQFPDAVFWQEIGEIFRQLQKQAAEIYNQSLIELYYEIFIKGKGFANASSVEHYLSDVCYTRAAELFKNAAIASGLRGKVKSNFRLKELKNMKSGLPTTKSDNFPIPLVKQKGGQYTGFEVSNHNSDFIIKIPFGRWQVKEEIDKYRPWEKFDFEQVRKNPKPISLLLSTQRRKRNKGWSKDEGTEAEIRKVMNGDYQTSYIEVKRGSKIGEKSAWMLNLSIDVPKIDKGVDPSIIGGIDVGVKSPLVCAINNALSRYSISDNDLFHFNKKMFARRRILLRRNRHKRAGHGARNKLKPITVLTEKSGRFRKKLMERWACEIANFFIKNKVGTVQMENLESMKRREDSYFNIRLRGFWPYAEMQSKIEFKLRQYGIEVRKVAPNNTSKTCSKCGHLNNYFNFEFRKKNKFPHFKCEKCNFKEDADYNAALNISNPKLKSTKEEP

SEQ ID NO: 1512 - protein, 726 aa, synthetic construct
SEVEFSHEYWMRHALTLAKRARDEREVPVGAVLVLNNRVIGEGWNRAIGLHDPTAHAEIMALRQGGLVMQNYRLTDATLYATFEPCVMCAGAMIHSRIGRVVFGVRNSKHGAAGSLMNVLNYPGMNHRVEITEGILADECAGLLCDFYRMPRQVFNARKKAQPSINPGGSSGGSSGSETPGTSESATPESSGGSSGGSAKNTITKTLKLRIVRPYNSAEVEKIVADEKNNREKIALEKNKDKVKEACSKHLKVAAYCTTQVERNACLFCKARKLDDKFYQKLRGQFPDAVFWQEIGEIFRQLQKQAAEIYNQSLIELYYEIFIKGKGFANASSVEHYLSDVCYTRAAELFKNAAIASGLRGKVKSNFRLKELKNMKSGLPTTKSDNFPIPLVKQKGGQYTGFEISSHNDDFIIKIPFGRWQVKKEIDKYRPWEKFDFAQVRKSPKPISLLLSTQRRKRNKGWSNDEGTEAEIRKVMNGDYQTSYIEVKRGSKIGEKSAWMLSLSIDVPRIDKGVDPSIIGGIDVGVKSPLVCAINNAFGRYSISDNDLFHFNKKMFARRRILLKKNRHKRAGHGAKNKLKPITILTEKSKRFRKKLIERWACEIADFFIKNKVGTVQMENLESMKRKEDSYFNIRLRGFWPYAEMQNKIEFKLKQYGIEIRKVAPNNTSKTCSKCGHLNNYFNFEYRRKNKFPHFKCEKCNFKENADYNAALNISNPKLKSTKEEP

SEQ ID NO: 1513 - protein, 726 aa, synthetic construct
SEVEFSHEYWMRHALTLAKRARDEREVPVGAVLVLNNRVIGEGWNRAIGLHDPTAHAEIMALRQGGLVIQNYRLSDATLYVTFEPCVMCAGAMIHSRIGRVVFGVRNSKRGAAGSLMNVLNYPGMNHCVEITEGILVDECAALLCDFYRMPRQVLSAQKKAQSSISSGGSSGGGSSSETPGASGSVTPKSSVGSSAGSTKNTITKTLKLRIVRPYNSAEVEKIVADEKNNREKIALEKNKDKVKEACSTHLKVAAYCTTQVERNACLFCKARKLDDKFYQKLRGQFPDAVFWQELGEIFRQLQKQAAEIYNQSLIELYYEIFIKGKGFANASSVEHYLSDVCYTRAAELFRNAAIASGLRGKVKSNFRLKELKNMKSGLPTTKSDNFPIPLVKQKGGQYTGFEISSHNDDFIIKIPFGRWQVKKEIDKYRPWEKFDFEQVRKSPKPISLLLSTQRRKRNKGWSKDEGTEAEIRKVMNGDYQTSYIEVKRGSKIGEKGAWMLNLSIDVPKIDKDVDPSIIGGIDVGVKSPLVCAIDNAFSRYSISDNDLFHFNKKMFARRRILLKKNRHRRAGHGAKNKLKPIAVLAKKSEGFRKKLIERWACEVADFFIKNKVGTVQMENLESMKRREDSYFNIRLRGFWPYAEMQNKIEFKLRQYGVEIRKVAPNNTSKTCSKCGHLNNYFDFEYRKKNKFPHFKCEKCNFKENADYNAALNISNPKLRSTKEEP

SEQ ID NO: 1514 - protein, 726 aa, synthetic construct
SEVEFSHEYWMRHALTLAKRARDEREVPVGAILVLNNRVIGEGWNRAIGLHDPTAHAEIMALRQGGLVMQNYRLTDATLYVTFEPCVMCAGAMIHSRIGRVVFGVRNSKRGAAGSLMNVLNYPGMNYCVEITEGILVDECAALLSDFYRMPRQVLNAQKKAQSSISSGGSSGGSSGSETPGASESVTPKSSGGSSGGSAKNTITKTLRLRIVRPYNSAEVEKIVADEKNNREKVALEKNKDKVREACSKHLKVAAYCTTQVERNACLFCKARRLDDKFYQKLRGQFPDAVFWQEIGEIFRQLQKQAAEIYNRSLIELYYEIFIKGKGIANASSVEHYLSDVCYTRAAELFKNAAIASGLRGKVKGNFRLKELKSMKSGLPTTKSDNFPIPLVKQKGGQYTGFEISSHNDDFIIKIPFGRWQVKKEIDRYRPWEKFDFEQVRKSPKPISLLLSTQRRKRNKGWSKDEGTEAEIRRVMNGDYQTSYIEVKRGSKVGEKSAWMLNLSIDVPKIDKGVDPSIVGGIDVGVKSPLVCAINNSFSRYSICDNDLFRFNKKMFARRRILLKKNRHKRAGHGAKNKLKPISVLTEKSGRFRKKLIERWACEITDFFIKNKVGTVQMENLGSMKRKEDSYFNIRLRGFWPYAEMQNKIEFKLKQYGIEIRKVAPDNTSKTCSKCGHLNNYFNFEYRKKNKFPHFKCEKCNFKEDADYNAALNISNPKLKSTKEEP

SEQ ID NO: 1515 - protein, 726 aa, synthetic construct
SEVEFSHEYWMRHALTLAKRARDEREVPVGAILVLNNRVIGEGWNRAIGLHDPTAHAEIMALRQGGLVMQNYRLIDATLYVTFEPCVMCAGAMIHSRIGRVVFGVRNNKHGAAGSLVNVLNYPGMNHRVEITEGILADECAALLCDFYRMPRQVFNARKKAQSSINPGGSSGGSSGSETPGTSESATPESSGGSSGSSTKNTITKTLKLRIVRPYNSAEVEKIVADEKNNREKIALEKNKDKVKEACSKHLKVAAYCTTQVGRNACLFCKARRLDDKFYQKLRGQFPDAVFWQEIGEIFRQLQKQAAEIYNQSLIELYYEIFIKGKGFANASSVEHYLSDVCYTRAAELFKNAAIASGLRGKVKSNFRLKELKNMKSGLPTTKSDNFPIPLVKQKGGQYTGFEISSHNDDFIIKIPFGRWQVKKEIDKYRPWEKFDFEQVRKSPKPISLLLSTQRRKRNKGWSKDEGTEAEIRKVMNGDYQTSYIEVKRGSKTGEKSAWMLNLSIDVPKIDKGVDPSIIGGIDVGVKSPLVCAINNAFSRYSISDNDLFRFNKKMFARRRILLGKNRHKRAGHGVKNKLKPITILTEKSGRFRKKLIERWACEIADFFIKNKVGTVQMENLESMKRKEDSYFNIRLRGFWPYAEMQNKIEFKLKQYGIEIRRVAPNNTSKTCSKCGHLNNYFNFEYRKKNKFPHFKCEKCNFKENADYNAALNISNPKLKSTKEEP

SEQ ID NO: 1516 - protein, 726 aa, synthetic construct
SEVEFSHEYWMRHALMLAKRARDEREVPVGAVLVLNNRVIGEGWNRAIGLHDPTAHAEIMALRQGGLAMQNYRLVDATLYVTFEPCVLCAGAMVHSRIGRVVFGVRNSKRGAAGSLMNVLNHPGMNHRVEITGGILADECAALLCDFYRMPRQVFNAQKKARSNINSGGSSGGSSGSETLGTSESATPESSGGSSGGSAKNTITKTLKLRIVRPYNSAEVEKIVADEKNNREKIALEKNKDKVKEACSEHLKVAAYCTTQVERNACLFCKARKLDDKFYQKLRGQFPDAVFWQEISEIFRQLQKQAAEIYNQSLIELYYEIFIKGKGFANASSVEHYLSDVCYTRAAELFKNAAIASGLRGKVKSNFRLKELKNMKSGLPTTKSDNFPIPLVKQKGGQYTGFEISSHNDDFIIKIPFGRWQVKKEIDKYRPWEKFDFEQVRKSPKPISLLLSTQRRKRNKGWSKDEGTEAEIRKVMNGDYQTSYIEVKRGSKIGEKSAWMLNLSIDVPKIDKGVDPSIIGGIDVGVKSPLVCAINNALSRYSISDNDLFHFNKKMFARRRILLRKNRHKRAGHGAKNKLKPITIMTEKSKRFRKKLIERWACEIADFFIKNKVGTVQMENLESMKRKEDSYFNVRLRGFWPYAEMQNKIEFKLKQYGIVVRKVAPNNTSKTCSKCGHLNNYFSFEYRKKNKFPHFKCEKCNFKEDADYNAALNISNPKLKSTKGEP

SEQ ID NO: 1517 - protein, 726 aa, synthetic construct
SEVEFSHEYWMRHALTLAKRARDEREVPVGAILVLNNRVIGEGWNRAIGLHDPTAHAEIMALRQGGLVMQNYRLIDATLYVTFEPCVMCAGAMIHSRIGRAVFGVRNSKHGAAGSLVNVLNYPGMNHRVEITEGILADECAALLCDFYRMPRQVFNARKKAQSSINPSGSSGGSSGSVTPGTSESATPESSGGGFGGSAKNTITKTLQLRIVRPYNSAEVEKIVADEKNNREKIALEKNKDKVKEACSKHLKVAAYCTTQVERNACLFCKARKLDDEFYQKLRGQFPDAVFWQEIGEIFRQLQKQAAEIYNQSLIELYYEIFIKGRGFANASSVEHYLSDVCYTRAAELFKNAAIASGLRGKVKSNFRLKELKNMKSGLPTTKSDNFPIPLVKQKGGQYTGFEISSHNDDFIIKIPFGRWQAKKEIDKYRPWEKFDFEQVRKSPKPISLLLSTQRRKRNKGWSKDEGTEAEIRKVMNGDYQTSYIEVKRGRKVGEKSVWMLNLSIDVPKIDKGVDPSTIGGIDVGVKSPLVCAINNAFSRYSISDNDLFRFNKKMFARRRILLKKNRHKRAGHGAKNKLKPITILAEKSGRFRKKLIERWACEIADFFIKNKVGTVQMENLESMKRKEDSYFNIRLRGFWPYAEMQNKIELKLKQHGIKIRKVAPNNTSKTCSKCGHLNDYFNFEYRKKNKFPHFKCEKCNFKEDADYNAALNISNPKLKSTRGEP

SEQ ID NO: 1518 - protein, 726 aa, synthetic construct
SEVEFSHEYWMRHALTLAKRARDEREVPVGAVLVLNNRVIGEGWNRAIGLHDPTAHAEIMALRQGGLVMQNYRLIDATLYVTFEPCVMCAGAMIHSRIGRVVFGVRNNKRGAAGSLMNVLNYPGMNHRVEITEGILADECAALLCDFYCMPRQVLNAQKKARSCINSGGSSGGSSSSETPGTSGSATPEGSVGSSGGSAKNTITKTLKLRIVRPYNSAEVEKIVADEKNNREKIALEKNKDKVKEACSKHLKVASYCTTQVERNACLFCKARKLDDKFYQKLRGQFPDAVFWQELGEIFRQLQKQAAEIYNQSLIELYYAIFIKGKGFANASSVEHYLSDVCYTRAAELFKNAAIASGLRGKVKSNFRLKELKNMKSGLPTTKSDNFPIPLVKQKGGQYTGFEISNHDGDFIIKIPFGRWQVKKEINKHRPWEKFDFEQVRKSPKPISLLLSTQRRKRNKGWSKDEGTEAEIRKVMNGDYQTSYIEVKRGSKIGEKSAWMLNLSIDVPKIDKGVDPGIIGGIDVGVKSPLVCAINNASSRYSISDNDLFHFNKKMFARRRILLKKNRHKRAGHGAKNKLKPITIMTEKSKRFRKKLIERWACEIADFFIKNKVGTVQMENLESMKRKEDSYFNIRLRGFWPYAEMQNKIEFKLKQYGIEVRRVAPNNTSKTCSKCGHLNNYFNFEYRKKNKFPHFKCEKCNFKEDADYNAALNISNPKLKSTKEEP

SEQ ID NO: 1519 - protein, 726 aa, synthetic construct
SEVEFSHEYWMRHALTLAKRARDEREVPVGAVLVLNNRVIGEGWNRAIGLHDPTAHAEIMALRQGGLVMQNYRLVDATLYVTFEPCVLCAGAMVHSRIGRVVFGVRNSKRGAAGSLMNVLNYPGMNHRVEITEGILADECAALLCDFYRMPRQVFIAQKKAQSSINPGGPSDGSSGSETPGTSESATPESSGDSSGGSAKNTITKTLKLRIVRPYNSAEVEKIVADEKNNREKIALEKNRDRVKEACSKHLKVAAYCTTQVERNACLFCKARRLDDKFYQKLRGQFPDAVFWQEIGEIFRQLQKQAAEIYNQSLIELYYEIFIKGKGFANASSVEHYLSDVCYTRAAGLFKNAAIASGLRGKVKSNFRLKELKNMKSGLPTTKSDNFPIPLVKQKGGQYTGFEISSHNDDFIIKIPFGRWQVKKEIDKYRPWEKFDFEQVRKSPKPISLLLSTQRRKRNKGWSKDEGTEAEIRKVMNGDYQTSYIEVKRGSKIGEKSAWMLNLSIDVPKIDKGVDPSIIGGIDVGVKSPLVCAINNALSRYSISDNDLFHFNKKMFARRRILLRKNRHKRAGHGARNKLKPISILTEKSKRFRKTLIERWACEIADFFIKNKVGTVQIENLESMKRKEDSYFNIRLRGFWPYAEMQNKIEFKLKQYGIKVRKVAPNNTSKTCSKCGHLNNYFSFEYRKKNKFPHFKCEKCNFKENADYNAALNISNPKLKSTKEEP

SEQ ID NO: 1520 - protein, 726 aa, synthetic construct
SEVEFSHEYWMRHALTLAKRARDEREVPVGAVLVLNNRVIGEGWNRAIGLHDPTAHAEIMALRQGGLVMQNYRLIDATLYVTFEPCVMCAGAMVHSRIGRVVFGVRNSKRGAAGSLTNVLDYPGMGHRVEITEGILADECAALLCDYYRMPRQVFNARKKAQSSINSGGSSDGGSDSETPGTSESATPESSGGSSGGSAKNTITKTLKLRIVRPYNSAEVEKIVADEKNNREKIALEKNKDKVKEACSKHLKVAAYCTTQVERNACLFCKARKLDDKFYQKLRGQFPDAVFWQEIGEVFRQLQKQAAEIYNQSLIELYYEIFIKGKGFANASSVEHYLSDVCYTRAAELFKNAAIASGLRGKVKGNFRLKELKNMKSGLPTTKSDNFPIPLVKQKGGQYTGFEISSHNDDFIIKIPFGRWQVKKEINKFRPWEKFDFEQVRKSPKPISLLLSTQRRKRNKGWSRDEGTEAEIRKVMNGDYQTSYIEVKRGSKIGEKSAWMLNLSIDVPKIDKGVDPSIIGGIDVGVKSPLVCAINNAFSRYSISDNDLFHFNKKMFARRRILLKKTRHKRAGHGAKNKLKPISILTGKSERFRKKLIERWACEIADFFIKNKVGTVQMENLESMKRKEDSYFNIRLRGFWPYAEMQNKIEFKLKQYGIEIRKVAPNNTSKTCSKCGHLNNYFNFEYRKKNKFPHFKCEKCNFKENADYNAALNISNPKLKSTKEKP

SEQ ID NO: 1521 - protein, 726 aa, synthetic construct
SEVEFSHEYWMRHALTLAKRARDEREVPVGAILVLNNRVIGEGWNRAIGLHDPTAHAEIMALRQGGLVMQNYRLTDATLYVTFEPCVMCAGAMIHSRIGRVVFGVRNNKHGAAGSLVNVLNYPGMNHRVETTEGILADECAALLCDFYRMPRQVFNARKKAQSSISPGGSSGGSSGSETPGTSESATLESSGGSSGGSAKNTITKTLKLRIVRPYNSAEVEKIVADEKNNREKIALEKNKDKVKEACSKHLKVASYCTTQVERNACLFCKARKLDDKFYQKLRGQFPDAVFWQEIGEIFRQLQKQAAEIYNQSLIELYYEIFIKGKGFANASSVEHYLSDVCYTRAAELFKNAAIASGLRGKVKSNFRLKELKNMKSGLPTTKSDNFPIPLVKQKGGQYTGFEISSHNDDFIIKIPFGRWQVKKEIDKYRPWEKFDFERVRKSPKPISLLLSTRRRKRNKGWSKDEGTEAEIRKVMNGDYQTSYIEVKRGSKIGEKSAWMLNLSIDVPKIDKGVDPSIIGGIDVGVKSPLVCAINNSSSRYSICDNDLFRFNKKMFARRRILLKKSRHKRAGHGAKNKLKPISILTEKSERFRKKLVERWACEIADFFIKNKVGTVQMENLEGMKRKEDSYFNIRLRGFWPYAEMQSKIEFKLKQYGIKIRKVAPNNTSKTCSKCGHLNNYFNFEYRKKNKFPHFKCEKCSFKENADYNAALNISNPKLKCTKEEP

SEQ ID NO: 1522 - protein, 726 aa, synthetic construct
SEVELSHEYWMRHALTLAKRARDEREVPVGAVLVLNNRVIGEGWNRAIGLHDPTAHAEMMALRQGGLVMQNYRLIDATLYVTFEPCVMCAGAMIHSRIGRVVFGVRNNRHGAAGSLVNVLDYPGMNHRVEITEGILADECAALLCDFYRMPRQVFNARKKAQSSISPGGSSGGSSGNETPGTSESATPESSGGSSGGSAKNTITKTLKLRIVRPYNSAEVEKIVADEKNSREKIALEKNKDKVKEACSKHLKVAAYCTTQVERNACLFCKARKLDDKFYQKLRGQFPDAVFWQEIGEVFRQLQKQAAEIYNQSLIELYYEIFIKGKGFANASSVEHYLSDVCYTRAAELFKNAAIASGLRGKVKSNFKLKELKSMKSGLPSTKSDNFPIPLVKQKGGQYTGFEISSHNDDFVIKIPFGRWQVKKEIDKYRPWEKFDFEQVRKSPKPISLLLSTQRRKRNKGWSKDEGTEAEIRKVMNGDYQTSYIEVKRGGKIGEKSAWMLSLSIDVPKIDKGVDPSIIGGIDVGVKSPLVCAINNTIGRYSISDNDLFRFNKKMFARRRILLKKNRHKRAGHGAKNKLKPISILTEKSGRFRKKLIERWACEIADFFIKNKVGTVQMENLESMKRKEDSYFNIRLRGFWPYAEMQNKIEFKLRQYGIEIRKVAPNNTSKTCSKCGHLNNYFSFEYRKKNKFPHFKCEKCNFKENADYNAALNISNPKLKSTKEEP

SEQ ID NO: 1523 - protein, 726 aa, synthetic construct
SEVEFSHEYWMRHALTLARRARDEREVPVGAVLVLNNRVIGEGWNRAIGLHDPTAHAEIMALRQGGLVMRNYRLIDATLYVTFEPCVMCAGAMIHSRISRVVFGVRNSKRGAAGSLMNVLNYPGMNHRVGITEGILADECAALLCDFYRMPRRVLNAQKKAQSSINSGGSSGGSSGSETPSTSESATPESSGGSSAGSTKNTITKTLKLRIVRPYNSAEVEKIVADEKNSREKIALEKNKDKVKEACSKHLKVAAYCTTQVERNACLFCKARKLDDKFYQKLRGQFPDAVFWQEVGEIFRQLQKQAAEIYNQSLIELYYEIFIKGKGFANASSVEHYLSDVCYTRAAELFKNAAIASGLRGKVKSNFRLKELKNMKSGLPTTKSDNFPIPLVKQKGGQYTGFEISNRNSDFIIKIPFGRWQVKKEINKYRPWEKFDFEQVRKSPKPISLLLSTQRRKRNKGWSKDEGTEAEIRKVMNGDYQTSYIEVKRGSRIGEKSAWMLNLSIDVPKVDKGVDPSIIGGIDVGVKSPLVCAINNAFSRCSISDNDLFRFNKKMFARRRILLKKNKHKRAGHGTKNKLKPITILTEKSRRFRKKLIERWACEIADFFIKNKVGTVQMESLESMKRKEDSYFNIRLRGFWPYAEMQNKIEFKLKQYGIKIRKVAPNNTSKTCSKCGHLNNYFSFEYRKKNKFPHFKCEKCNFKENADYNAALNISNPKLMSTKVEP

SEQ ID NO: 1524 - protein, 726 aa, synthetic construct
GEVEFSHEYWMRHALALAKRARDEREVPVGAILVLNNRVIGEGWNRAIGLHDPTAHAEIMALRQGGLVLQNYRLIDATLYVTFEPCVMCAGAMIHSRIGRVVFGVRNNKHGAAGSLVNVLNYPGMNHRVEITEGILANECAALLCDFYRMPRQVFNARKKAQSSINPGGSSGGRSGSETPGTSESATPESSGGSSGGSAKNTITKTLKLRIVRPYNSAEVEKIVADEKNNREKIALEKNKDKVKEACSKHLKVASYCTTQVERNACLFCKARKLDDKFYQKLRGQFPDAVFWQELGEIFRQLQKQAAEIYNQSLIELYYEIFIKGKGFANASSVEHYLSDVCYTRAAELFKNAAIASGLRGKVKSNFRLKELKNMKSGLPTTKSDNFPIPLVKQKGGQYTGFEISSHNDDFIIKIPFGRWQVKKEIDKYRPWEKFDFEQVRKSPKPISLLLSTQRRKRNKGWSRDEGTEAEIRKVMNGDYQTSYIEVKRGSKVGEKSAWMLNLSIDVPKIDKGVDPSIIGGIDVGVKSPLVCAINNAFSRYSISDNDLFHFNKKMFARRRILLKKTRHKRAGHGAKNKLKPISILTEKSERFRKKLIERWACEIADFFIKNKVGTVQMENLESMKRREDSYFNIRLRGFWPYAKMQNKIEFKLKQYGIEIRKVAPNNTSKTCSKCGHLNNYFNFEYRKKNKFPHFKCEKCNFKESADYNAALNISNPKLKSTKEEP

SEQ ID NO: 1525 - protein, 726 aa, synthetic construct
SEVEFSHEYWMRHALTLAKRARDEREVPVGAILVLNNRVIGEGWNRAIGLHDPTAHAEIMALRQGGLVMQNYRLIDATLYVTFEPCVMCAGAMIHSRIGRVVLGVRNNKHGAAGSLVNVLDYPGMNHRVEITEGILADECAALLCDFYRMPRQVFNARKKAQSSISPGGSSGGSSGSETPGTSESATPESSGGSSGGSAKNTITKTLKLRIVRPYNSAEVEKIVADEKNNREKIALEKNKDKVKEACSKHLKVASYCTTQVERNACLFCKARKLDDKFYQKLRGQFPDAVFWQEIGEVFRQLQKQAAEIYNQSLIELYYKIFIKGKGFANASSVEHYLSDVCYTRAAELFKNAAIASGLRGKVKSNFRLKELKNMKSGLPTTKSDNFPIPLVKQKGGQYTGFEIGSHNDDFIIKIPFGRWLAKKEIDKYRPWEKFDFEQVRKSPKPISLLLSTQRRKRNRGWSKDEGTEAEIRKVMNGDYQTSYIEVKRGSKIGEKSAWMLNLSIDVPKIDKGVDPSIIGGIDVGVKSPLVCAINNAFSRYSISDNDLFRFNKKVFARRRILLKKNRHKRAGHGTKNKLKPITILTEKSGRFRKKLIERWACEIANFFIKNKVGTVQMENLESMKRKEDSYFNIRLRGFWPYAEMQNKIEFKLKQYGIKIRKVAPNNTSKTCSKCGHLNNYFSFEYRKKNKFPHFKCEKCNFKEDADYNAALNISNPKLKSTKEEP

SEQ ID NO: 1526 - protein, 726 aa, synthetic construct
SEVEFSHEYWMRHALTLAKRARDEREVPVGALLVLNNRVIGEGWNRAIGLHDPTAHAEIMALRQGGLVMQNYRLTDATLYVTFEPCAMCAGAMIHSRIGRVVFGVRNSKHGAAGSLMNVLNYPGMNHRVEITEGILADECAALLCDFYRMPRQVFNARKKAQSSINPGGPSGGSSGSETPDTSESTTPESSGGNSGGSAKNTITKTLKLRIVRPYNSAEVEKIVADEKNNREKIALEKNKDKVKEACSEHLKVAAYCTTQVERNACLFCKARKLDDKFYQKLRGQFPDAVFWQELGEIFRQLQKQTAEIYNQSLIELYYEIFIKGKGFANASSVEHYLSDVCYTRAAELFKNAAIASGLRGKVKGNFRLKELKNVRSGLPTTKSDNFPIPLVKQKGGQYTGFEISSHNDDFIIKIPFGRWQAKKEIDKYRPWEKFDFEQVRKSPKPISLLLSTQRRKRNKGWSKDEGTEAEIRKVMNGDYQTSYIEVKRGSKIGEKSAWMLNLSIGVPKIDKGVDPSIIGGIDVGVKSPLVCAINNDFGRYSISDNDLFHFNKKMFARRRILLKKNRHKRAGHGAKNKLKPISVLTEKSGRFRKKLIERWACEIADFFIKNKVGTVQMENLGSMKRKEDSYFNIRLRGFWPYAEMQNKIEFKLKQYGIEIRKVAPDNTSKTCSKCGHLNNYFNFEYRKKNKFPHFKCEKCNFKEDADYNAALNISNPKLKSTKGEP

SEQ ID NO: 1527 - protein, 726 aa, synthetic construct
SEVEFSHEYWMRHALTLAKRARDEREVPVGAILVLNNRVIGEGWNRAIGQHDPTAHAEIMALRQGGLVMQNYRLINATLYVTFEPCVMCAGAMIHSRIGRVVFGVRNSKHGAAGSLMNVLNYPGMNHRVEITEGILADECAALLCDFYRMPRQVFSARKKAQSSINSGGSSGGNSGSKTPGTSESATPESSGGGSSGSAKNTVTKTLQLRIVRPYNSAEVEKIVADEKNNREKIALEKNKDKVKGACSRHLKVASYCTTQVERNACPFCKARKLDDKFYQKLRGQFPDAVFWQELGEIFRQLQKQAAEIYNQSLIELYYEIFIKGKGFANASSVEHYLSDVCYTRAAELFKNAAIASGLRGRVKSNFRLKELKNMKSGLPTTKSDNFPIPLVKQKGGQYTGFEISSHNDDFIIKIPFGRWQVKKEIDKYRPWEKFDFEQVRKSPKPISLLLSTQRRKRNKGWSKDEGTEAEIRKVMNGDYQTSYIEVKRGSKIGEKSAWMLSLSIDVPRIDKGVDPSIIGGIDVGVKSPLVCAINNALSRYSISDNDLFHFNKKMFARRRILLKKNRHRRAGHGAKNKLKPITILTEKSKRFRKKLIERWACEIADFFIKNKVGTVQMENLESMKRKEDSYFNIRLRGFWPYAEMQNKIEFKLKQYGIEIRRVAPNNTSRTCSKCGHLNNYFNFEYRRKNKFPHFKCEKCNFKEDADYNAALNISNPKLKSTKEEP

SEQ ID NO: 1528 - protein, 726 aa, synthetic construct
SEVEFSHEYWMRHALTLAKRARDEREVPVGAVLVLNNRVIGEGWNRAIGLHDPTAHAEIMALRQGGLVMQNHRLVDATLYVTFEPCVMCAGAMVHSRVGRVVFGVRNSKRGAAGSLMNVLDYPGMGHRVEITEGILADECAALLCDFYCMPRQVFNAQKRAQSSINPGGSSGGSSGSETPGASGSVTPKSSGGSSAGSTKGTITKTLKLRIVRPYNSAEVEKIVADEKNNREKIALEKNKDKVKEACSEHLKVAAYCTTQVERNACPFCKARKLDDKFYQKLRGQFPDAVFWQEIGEIFRQLQKQAAEIYNRSLIELYYEIFIKGKGIANASRVEHYLSDVCYTRAAELFKNAAIASGLRNRIKSNFRLKELKNMKSGLPTTKSDNFPIPLVKQKGGQYTGFEISNHNSDFIIKIPFGRWQAKKEIDKYRPWEKFDFEQVRKSPKPISLLLSTQRRKRNRGWSKDEGTEAEVKKVMNGDYQISYIEVKRGSKIGEKSAWTLNLSIDVPKIDKGVDPSIIGGIDVGVKSPLVCAISNALSRYSINDNDLFHFNKKMFARRRILLKKNRRRRAGHGAKNKLKPITILTEKSVRFRKKLIERWACEIADFFIKNKVGTVQMENLESMKRKEDSYFNIRLRGFWPYAEMQNKIEFKLKQYGIEIRRVAPNNTSRTCSKCGHLNNYFNFEYRRKYKFPHFKCEKCNFKEDADYNAALNISNPKLKSTKEEP

SEQ ID NO: 1529 - protein, 726 aa, synthetic construct
SEVEFSHEYWMRHALTLAKRARDEREVPVGAILVLNNRVIGEGWNRAIGLHDPTAHAEIMALRQGGLVMQNYRLIDATLYVTFEPCVMCAGAMIHSRIGRVVFGVRNNKHGAAGSLVNVLNYPGMNHRVEITEGILADECAALLCDFYRMPRQVFNARKKAQSSINPGGSSGGSGGSETPGTSESATPENSGGSSGSSAKNTITKTLKLRIVRPYNSAEVEKIVADEKNNREKIALEKNKDKVKEACSKHLKVASYCTTQVERSACPFCKARKLDDKFYQKLRGQFPDAVFWQELGEILRQLQKQAAEIYNQSLVELYYEILIKSKGIANASSVEHYLSDVCYTRAAELFKNAAIASGLRNKIKSNFRLKELRNMKSGLPTTKSDNFPIPLVKQKGGQYTGFEISSHDDDFIIKIPFGRWQVKKEIDKYRPWEKFDFEQVRKSPKPISLLLSTRRRKRNKGWSKDEGTEAEIRKVMNGDYQTSYIEVKRGSKIGEKSAWMLNLSIDVPKIDKGVDPSIIGGIDVGVKSPLVCAINNAFSRYSISDNDLFHFNKKMFARRRILLKKNRHKRAGHGAKNKLKPISILTEKSGRFRKKLIERWACEIADFFIKNKVGTVQMENLESMKRKEDSYFNIRLRGFWPYAEMQNKIEFKLKQYGIEIRKVAPNNTSKTCSKCGHLNSYFNFEYRKMNKFPHFKCEKCNFKENADYNAALNISNPKLKSAKEEP

SEQ ID NO: 1530 - protein, 726 aa, synthetic construct
SEVEFSHEYWMRHALTLAKRARDEREVPVGAVLVLNNRIIGEGWNRAIGLHDPTAHAEIMALRQGGLVMQNYRLVDATLYVTFEPCVLCAGAMVHSRIGRVVFGVRNSKRGAAGSLMNVLNYPGMNHRVEVTEGILADECAALLCDFYRMPRQVFNAQKKARSNINSGGSSGGSSGSETPGTSESATPESSGGSSAGSTKDTITKTLKLRIVRPYNSAEVEKVVADEKNNREKIAMEKNKDKVKEACSKHLKVASYCTTQVERNACLFCKARKLDDKFYQKLRGQFPDAVFWQELGGIFRQLQKQAAEIYNQSLIELYYEIFIKGKGFANASSVEHYLSDVCYTRAAELFKNAAIASGLRGKVKSNFRLKELKNMKSGLPTTKSDNFPIPLVKQKGGQYTGFEISSHNDDFVIKIPFGRWQVKKEIDKYRPWEKFDFEQVRKSPKPISLLLSTQRRKRNKGWSKDEGTEAEIRKVMSGDYQTSYIEVKRGSKTGEKSAWMLSLSIDVPKIDKGVDPSIVGGIDVGVKSPLVCAINNALSRYSISDNDLFHFNKKMFARRRILLRKNRHKRAGHGAKNKLKPITILTEKSMRFRKKLIERWACEIADFFIKNKVGTVQMENLESMKGKEDSYFNIRLRGFWPYAEMQNKIEFKLKQYGIVVRKVAPNNTSKTCSKCGHLNNYFNFEYRKKNKFPHFKCEKCNFKEDADYNAALNISNPKLKSTKGEP

SEQ ID NO: 1531 - protein, 726 aa, synthetic construct
SEVEFSHEYWMRRALTLAKRARDEREVPVGAVLVLNNRVIGEGWNRAIGLHDPTAHAEIMALRQGGLVIQNYRLSDATLYVTFEPCVMCAGAMIHSRIGRVVFGVRNSKRGAAGSLMNVLNYPGMNHCVEITEGILVDECAALLCDFYRMPRQVLSAQKKAQSSISSGGSSGGSSGSETPGASGSVTPKSSVGSSAGSTKNTITKTLKLRIVRPYNSAEVEKIVADEKNNREKIALEKNKGKVREACSKHLEVAAYCITQVERNACLFCKARKLDDKFYQKLRGQFPDAVFWQELGEIFRQLQKQAAAIYNQSLIELYYEIFIKGKGFANASSVEHYLSDVCYTRAAELFKNAAIASGLRGKVKSNFRLKELKNMKSGLPTTKSDNFPIPLVRQKGGQYTGFEISSHNDDFVIKIPFGRWQVKKEIDKYRPWEKFDFEQVRKSPKPISLLLSTQRRKRNRGWSKDEGTEAEIRKVMNGDYQTSYIEVKRGGKIGEKSAWMLNLSIDVPKIDKGVDPSTIGGIDVGVKSPLVCAINNAFCRYSISDNDLFHFNKKMFARRRILLKKSRHKRAGHGAKNKLKPISILTEKSKRFRKKLIERWACEIADFFIKNKVGTVQMENLESMKRKEDSYFNIRLRGFWPYAEMQNKIEFKLKQYGIEIRKVAPNNTSKTCSKCGHLNNYFNFEYRKKNKFPHFKCEKCNFKENADYNAALNISNPKLKSTKEEP

SEQ ID NO: 1532 - protein, 726 aa, synthetic construct
SEVEFSHEYWMRHALTLAKRARDEREVPVGAILVLNNRVIGEGWNRAIGLHDPTAHAEIMALRQGGLVMQNYRLIDATLYVTFEPCVMCAGAMIHSRIGRVVFGVRNSKHGAAGSLVNVLNYPGMNHRVEITEGILADECAVLLCDFYRMPRQVFNARKKAQSSINPGGSSGGSSGSVTPGTSESATPESSGGGFGGSAKNTITKTLKLRIVRPYNSAEVEKIVADEKNNREKIALERNKGKVKEACSKHLKVAAYCTTQVERNACLFCKARKLDDKFYQKLRGQFPDAVFWQEIGEIFRQLQKQAAEIYNQSLIELYYEIFIKGKGFANASSVEHYLSDVCYTRAAELFKNAAIASGLRGKVKSNFRLKELKNMRSGLPTTKSDNFPIPLVKQKGGQYTGFEISNHDGDFIIKIPFGRWQVKKEINKHRPWEKFDFEQVRKNPKPISLLLSTQRRKRNKGWSKDEGTEAEIRKVMNGDYQTSYIEVKRGSKIGEKSVWMLNLSIDVPKIDKGVDPSIIGGIDVGVKSPLVCAINNALSRYSISDNDLFHFNKKMFARRRILLRKNRHKRAGHGAKNKLKPITTMTEKSKRFRKKLIERWACEIADFFIKNKVGTVQMENLESMKRREDSYFNIRLRGFWPYAEMQNKIEFKLRQYGIEIRKVAPNNTSKTCSKCGHLNNYFDFEYRKKNKFPHFKCEKCNFKENADYNAALNISNPKLRSTGEEP

SEQ ID NO: 1533 - protein, 726 aa, synthetic construct
SEVEFSHEYWMRHALTLAKRARDEREVPVGAILVLNNRVIGEGWNRAIGLHDPTAHAEIMALRQGGLVMQNYRLIDATLYVTFEPCVMCAGAMIHSRIGRVVFGVRNNKHGAAGSLVNVLNYPGMNHRVEITEGILADECAALLCDFYRMPRQVFNARKKAQSSINPGGSSGSSSGSETPGTSESATPESSGGSSGGSAKNTITKTLKLRIVRPYNSAEVEKIVADEKNNREKIALEKNKGKVKEACSKHLKVAAYCTTLVERNACLFCKARRLDDKFYQKLRGQFPDAVFWQEIGEIFRQLQKQAAEIYNQSLIELYYEIFIKGKGFANASSVEHYLSDVCYTRAAELFKNAAIASGLRGKVKSNFRLKELKNMRSGLPTAKSDNFPIPLVKQKGGQYTGFEISSHNDDFIIKIPFGRWQVKKEIDKYRPWEKFDFEQVRKSPKPISLLLSTRRRKRNKGWSKDEGTEAEIRKVMNGDYQTSYIEVKRGSKIGEKSAWMLNLSIDVPKVDKGVDPSIIGGIDVGVKSPLVCAINNAFSRYSISDNELFHFNKKMFARRRILLKKNRHKRAGHGAKNKLKPISVLTEKSGRYRKKLIERWACEIADFFIKNKVGTVQMENLGSMKRKEDSYFNIRLRGFWPYAEMQNKIEFKLKQYGIEIRKVAPDNTSKTCSKCGHLNNYFNFEYRKKNKFPHFKCERCNFKEDADYNAALNISNPKLKSTKEEP

SEQ ID NO: 1534 - protein, 726 aa, synthetic construct
SEVEFSHEYWMRHALTLAKRARDEREVPVGAILVLNNRVIGEGWNRAIGLHDPTAHAEIMALRQGGLVMQNYRLTDATLYVTFEPCVMCAGAMIHSRIGRVVFGIRNSKRGAAGSLMNVLNYPGMNHCVKITEGVLVDECAALLCDFYRMPRQVLSAQKKAQSSISSGGSSGGSSGSETPGASESATPKSSGGSSAGSTRDTITKTLKLRIVRPYNSAEVEKIVADEKNSREKIALEKNKDKVKEACSEHLKVAAYCTTQVERNACLFCKARKLDDGFYQKLRGQFPDAVFWQEIGEIFRQLQKQAAEIYNQSLIELYYEIFIKGKGFANASSVEHYLSDVCYTRAAGLFKNAAIASGLRGKVKSNFRLKELKNMKSGLPTTKSDNFPIPLVKQKGGQYTGFEISNHNDDFIIKIPFGRWQVKKEIDKYRPWEKFNFEQVRKSPKPISLLLSTQRRKRNKGWSKDEGTEAEIKKVMNGDYQTSYIEVKRGSKIGEKSAWMLNLSINVPKIDKGVDPSIIGGIDVGVKSPLVCAINNAFSRYSISDNDLFHFNKKMFARRRVLLKKNRHRRAGHGAKNKLKPITILTEKSVRFRKKLIERWACEIADFFIKNKVGTVQMENLESMKRKEDSYFNIRLRGFWPYAEMQNKIEFKLKQYGIEIRRVAPNNTSRTCSKCGHLNNYFNFEYRKKNKFPHFKCEKCNFEENADYNAALNISNPKLKSTKEEP

SEQ ID NO: 1535 - protein, 726 aa, synthetic construct
SEVEFSHEYWMRHALTLAKRARDEREVPVGAILVLNNRVIGGGWNRAIGLHDPTAHAEIMALRQGGLVTQNYRLIDATLYVTFEPCVMCAGAMIHSRIGRVVFGVRNSKHGAAGSLVNVLNYPGMNHHVEITEGILADECAALLCDFYRMPRQVFNARKKAQSSINPGSSSGGSSGSETPGTCESATPESSGGSSGGSAKNTITKTLKLRIVRPYNSAEVEKIVADEKNNREKIALEKNKDKVKEACSKHLKVAAYCTTQVERSACLFCKARRLDDKFYQKLRGQFPDAVFWQELGEIFRQLQKQAAEIYNQSLIELYYEIFIKGKGITNASRVEHYLSDVCYTRAAELFKNAAVASGLRSKVRSNFRLKELKNMKSGLPTTKSDNFPIPLVKQKGGQYTGFEISSHNSDFIIKIPFGRWQVKEEIDKYRPWEKFDFEQVRKSPKPISLLLSTQRRKRNKGWSKDEGTEAEIRKVMNGDYQTSYIEVKRGSKIGEKSAWMLNLSIDVPKIDKGVDPGIIGGIDVGVKSPLVCAINNASSRYSISDNDLFHFNKKMFARRRILLKKNRHKRAGHGAKNKLKPITIMTEKSKRFRKKLIERWACEIADFFIKNKVGTVQMENLESMKRKEDSYFNIRLRGFWPYAEMQNKIEFKLKQYGIEIRRVAPNNTSRTCSKCGHLNNYFNFEYRKKNKFPHFKCEKCNFKENADYNAALNISNPKLKGTKEEP

SEQ ID NO: 1536 - protein, 726 aa, synthetic construct
SEDEFSHEYWMRHALTLAKRARDGREVPVGAVLVLNNRVIGEGWNRAIGLHDPTAHAEIMALRQGGLVMQNYRLIDATLYVTFEPCVMCAGAMVHSRIGRVVFGVRNSKRGAAGSLMNVLDYPGMGHRVEITEGILADECAALLCDFYCMPRQVLDAQKKAQSSISPGGSSGGSSGSETPGASGSVTPKSSGGSSAGSTKDTITKTLKLRIVRPYNSAEVEKIVADEKNSREKIALEKNKDKVKEACSEHLKVAAYCTTQVERNACLFCKARKLDDRFYQKLRGQFPDAVFWQEIGEIFRQLQKQAAEIYNQSLIELYYEIFIKGKGITNTSRVEHYLSDVCYTRAAELFKNAAIASGLRGKVKSNFRLKELKNMKSGLPTTKSDNFPIPLVKQKGGQYTGFEISSHNDDFIIKIPFGRWQVKKEIDKYRPWEKFDFEQVRKSPKPISLLLSTQRRKRNKGWSKDEGTEAEIRKVMNGDYQTSYIEVKRGSKIGEKSAWMLSLSIDVPKIDKGVDPSIIGGIDVGVKSPLVCAINNAFCRYSISDNDLFHFNKKMFARRRILLKKSRHKRAGHGAKNKLKPISILTEKSKRFRKKLIERWACEIADFFIKNKVGTVQMENLESMKRKEDSYFNIRLRGFWPYAEMQNKIEFKLKQYGIEIRKVAPNNTSKTCSKCGHLNNYFNFEYRKKNKFPHFKCEKCSFKENADYNAALNISNPKLKSTKEEP

SEQ ID NO: 1537 - protein, 726 aa, synthetic construct
SEVEFSHEYWMRHALTLAKRARDEREVPVGAILVLNNRVIGEGWNRAIGLHDPTAHAEIMALRQGGLVMQNYRLIDATLYVTFEPCVMCAGAMIHSRIGRVVFGVRNNKHGAAGSLVNVLNYPGMNHRVEITEGILADECAALLGDFYRMPRQIFNARKKAQSSINSGGPSGGSSGSETPGTSESATPESSGGSSGGSAKNTITKTLKLRIVRPYNSAEVEKIVADEKNSREKIALEKYKDKVKEACSKHLMVAPYCTTQVERNACLFCKARELDGKFYQKLRDQFPDAVFWQELGEIFRQLQKQAAEIYNRGLIELYYEIFVKGKGIANASSVEHYLSDVCYTRAAELFKNAAIASGLRNKIKSNFRLKELRNMKSGLPTTKSDNFPIPLVRQKGGQYTGFEISNHDGDFIIKIPFGRWQVKKETNKHRPWEKFDFEQVRKSPKPISLLLSTQRRKRNKGWSKDDGTEAEVRRVMNGDYQTSYIEVKRGSRIGEKSAWMLSLSIDVPKIDRGVDPSIIGGIDVGVKSPLVCAINNALSRYSISDNDLFHFNKKMFARRRILLKKNRHRRAGHGARNKLKPITVLTEKSKRFRKKLIERWACEIADFFIKNKVGTVQMENLESMKRKEDSYFNIRLRGLWPYAEMQNKIEFKLKQYGIEIRKVAPNNTSKTCSKCGHLNNYFNFEYRRKNKFPHFKCEKCNFKENADYNAALNICNPKLKGTKEEP

SEQ ID NO: 1538 - protein, 726 aa, synthetic construct
SEVEFSHEYWMRHALILAKRARDEREVPVGAVLVLNNRVIGEGWNRAIGLHDPTAHAEIMALRQGGLVMQDYRLIDATLYVTFEPCVMCAGAMVHSRIGRVVFGVRNSKRGAAGSLMNVLDYPGMGHRVEITEGILADECAALLCDFYCMPRQVFNAQKRAQSSINSGGSSGGSGGSETPGTSENATPGSSCGSSGGSAKNTITKTLKLRIVRPYNSAEVEKIVADEKNSREKIALEKNKDKVKEACSKHLKVAAYCTTQVERNACLFCKARKLDDRFYQKLRGQFPDAVFWQEIGEIFRQLQKQAAEIYNQSLVELYYEILIKGKGIANASSVEHYLSDVCYTRAAELFKNAAIASGLRNKIKSNFRLKELRNMKSGLPTTKSDNFPIPLVKQKGGQYTGFEISSHNGDFIIKIPFGRWQVKKEIDKYRPWEKFDFEQVRKSPKPISLLLSTQRRKRNKGWSKDEGTEAEIRKVMNGDYQTSYIEVKRGSKIGEKSAWMLNLSIDVPKIDKGVDPSIIGGIDVGVKSPLVCAINNAFSRYSICDNDLFRFNKKMFARRRILLKKNRHKRAGHGAKNKLKPISILTEKSERFRKKLIEKWACEIADFFIKNKVGTVQMENLESMKRREDSYFNIRLRGFWPYAEMQNKIEFKLKQYGIKVRKVAPNNTSKTCSKCGHLNNYFSFEYRKKNKFPHFKCEKCNFKENADYNAALNISNPKLKSTKEEP

SEQ ID NO: 1539 - protein, 726 aa, synthetic construct
SEVEFSHEYWMRHALTLAKRARDEREVPVGAVLVLNNRVIGEGWNRAIGLHDPTAHAEIMALRQGGLVMQNYRLTDATLYVTFEPCVMCAGAMIHSRIGRVVFGVRNSKHGAAGSLVNVLDYPGMNHSVEITEGILADECAALLCDFYRMPRQVFNARKKAQSSINPGGSSGGSSGSETPGTSESATPESSGGNSGGSAKNTITKTLQLRIVRPYNSAEVEKIVTDEKNNREKIALEKNKDKVKEACSKHLKMASYCTTLVERNACLFCKARKLDDKFYQKLRGQFPDAVFWQELGEIFRQLQKQAAEIYNQSLIELYYEIFIKGKGFANASSVEHYLSDVCYTRAAELFKNAAIASGLRGKVKSNFKLKELKNMKSGLPTTKSDNFPIPLVKQKGGQYTGFEISSHNDDFIVKIPFGRWQAKKEIDKYRPWEKFDFEQVRKSPKPISLLLGTQRRKRNKGWSKDEGTEAEIRKVMNGDYQTSYIEVKRGSKIGEKSAWMLSLSIDVPKIDKGVDPSIIGGIDVGVKSPLVCAINNAFSRYSISDNDLFHFNKKMFARRRILLKKNRHKRAGHGAKNKLKPISILTGKSERFRKKLIERWACEIADFFIKNKVGTVQMENLESMKRKEDSYFNIRLRGFWPYAEMQNKIEFKLKQYGIEIRKVAPNNTSKTCSKCGHLNNYFNFEYRKKNKFPHFKCEKCNFKENADYNAALNISNPKLKSTKGEP

SEQ ID NO: 1540 - protein, 726 aa, synthetic construct
SEVEFSHEYWMRHALTLAKRARDEREVPVGAVLVLNNRVIGEGWNRAIGLHDPTAHAEIMALRQGGLVMRNYRLTDATLYVTFEPCVMCAGAMIHSRIGRVVFGVRNSKRGAAGSLMNVLNYPGMNHCVEITEGILVDECAALLCDFYRMPRQVLNAQKKAQSSISPGGSSGGSSGSETPGASGSVTPKSSGGSSAGSTKDTITKTLKLRIVRPYNSAEVEKIVADEKNNREKIALEKNKDKVKEACSEHLKVAAYCTTQVERSACLFCKARKLDDKFYQKLRGQFPDAVFWQEIGEVFRQLQKQAAEIYNQSLIELYYEILIKGKGFANASSVEHYLSDVCYTRAAELFKNAAIASGLRGKVKSNFRLKELKNMKSGLPTTKSDNFPIPLVKQKGGQYTGFEISSHNDDFIIKIPFGRWQVKKEIDKYRPWEKFDFEQVRKSPKPISLLLSTQRRKRNKGWSKDEGTEAEIRKVMNGDYQTSYIEVKRGSKIGEKSAWMLNLSIDVPKIDKGVDPSIIGGIDVGVKSPLVCAINNAFSRYSICDNDLFRFNKKMFARRRILLGKNRHKRAGHGVKNKLKPITILTEKSGRFRKKLIERWACEIANFFIKNKVGTVQMENLESMKRKEDSYFNIRLRGFWPYAEMQNKIEFKLKQYGIEIRKVAPNNTSKTCSKCGHLNSYFDFEYRKKNKFPHFKCEKCNFKENADYNAALNISNPKLKSTKEEP

SEQ ID NO: 1541 - protein, 726 aa, synthetic construct
SEVEFSHEYWMRHALTLAKRARDEREVPVGAILVLNNRVIGEGWNRAIGLHDPTAHAEIMALRQGGLVTQNYRLIDATLYVTFEPCVMCAGAMIHSRIGRVVFGVRNSKHGAAGSLVNVLNYPGMNHRVEITEGILADECAALLCDFYRMPRQVFNARKKAQSSINPSGSSGGSSGSVTPGISESATPESSGGGFGGSAKNTITKTLQLRIVRPYNSAEVEKIVADEKNSREKIALEKNKDKVKEACSKHLKVASYCTTQVERNACLFCKARKLDDKFYQKLRGQFPDAVFWQELGEIFRQLQKQAAEIYNQSLIELYYEIFIKGKGLANASSVEHYLSDVCYTRAAELFKNAAIASGLRGKVKSNFKLKELKSMKSGLPSTKSDNFPIPLVKQRGGQYTGFEISSHNDDFIIKIPFGRWQAKKEIDKYRPWEKFDFEQVRKSPKPISLLLSTQRRKRNRGWSKDEGTEAEIRKVMNGDYQTSYIEVKRGSKIGEKSAWMLNLSIDVPKIDKGVDPSIIGGIDVGVKSPLVCAINNAFSRYSISDNDLFRFNKKMFARRRILLGKNRHKRAGHGVKNKLKPITILTEKSGRFRKKLIERWACEIADFFVKNKVGTVQMENLESMKRKEDSYFNIRLRGFWPYAEMQNKIEFKLKQYGIKVRKVAPNNTSKTCSKCGHLNNYFSFEYRKKNKFPHFKCEKCNFKENADYNAALNISNPKLKSTKEEP

SEQ ID NO: 1542 - protein, 726 aa, synthetic construct
SEVEFSHEYWMRHALTLAKRARDEREVPVGAVLVLNNRVIGEGWNRAIGLHDPTAHAEIMALRQGGLVMQNYRLIDATLYVTFEPCVMCAGAMIHSRIGRVVFGVRNSKHGAAGSLVNVLNYPGMNHRVEITEGILADECAALLCDFYRMPRQVFNARKKAQSSINPSGSSGGSSGSVTPGTSESATPESSGGGFGGSAKNTITKTLQLRIVRPYNSAEVEKIVADEKNNREKIALEKNKDKVKEACSKHLKVASYCTTQVERNACLFCKARKLDDKFYQKLRGQFPDAVFWQEIGEIFRQLQKQAAEIYNQSLIELYYEIFIKGKGIANASSVGHYLSDVCYTRAAELFKNAAIASGLRSKIKSNFRLKELRNMRGGLPTTKSDNFPIPLVKQKGGQYTGFEISSHNDDFIIKIPFGRWQVKKEIDKYRPWEKFDFEQVRKSPKPISLLLSTQRRKRNKGWSKDEGTEAEIRKVMNGDYQTSYIEVKRGSKIGEKSAWMLNLSIDVPKIDKGVDPSIIGGIDVGVKSPLVCAINNAFSRYSISDNDLFRFNKKVFARRRILLKKNRHKRAGHGTKNKLKPITILTEKSGRFRKKLIERWACEIANFFIKNKVGTVQMENLESMKRKEDSYFNIRLRGFWPYAEMQNKIEFKLKQYGIKVRKVAPNNTSKTCSKCGHLNNYFSFEYRKKNKFPHFKCEKCNFKENADYNAALNISNPKLKSTKEEP

SEQ ID NO: 1543 - protein, 726 aa, synthetic construct
SEVEFSHEYWMRHALTLAKRARDEREVPVGAVLVLNNRVIGEGWNRAIGLHDPTAHAEIMALRQGGLVMQNYRLIDATLYVTFEPCVMCAGAMVHSRIGRVVFGVRNSKRGAAGSLMNVLDYPGMDHRVEITEGILADECAALLCDFYRMPRQVLNAQKKAQSSINSGGSSGGSSSSETPGTSESATSESSGGGSSGSAKNTITKTLQLRIVRPYNSAEVEKIVADEKNSREKIALEKNKDKVKEACSKHLKVASYCTTQVERNACPFCKARKLDDKFYQKLRGQFPDAVFWQELGEILRQLQKQAAEIYNQSLIELYYEIFIKGRGFANASSVEHYLSDVCYTRAAELFKNAAIASGLRGKVKSNFRPKELKNMKSGLPTTKSDNFPIPLVKQKGGQYTGFEISSHNDDFIIKIPFGRWQVKKEIDKYRPWEKFDFEQVRKSPKPISLLLSTQRRKRNKGWSKDEGTEAEIRKVMNGDYQTSYIEVKRGSKTGEKSAWMLSLSIDVPKIDKGVDPSIIGGIDVGVKSPLVCAINNAFSRYSISDNDLFRFNKKMFARRRILLKKNRHKRAGHGAKNKLKPISILTRKSERFRRKLIERWACEIADFFIKNKVGTVQMENLESMKRKEDSYFNIRLRGFWPYAEMQNKIEFKLKQYGIEIRKVAPNNTSKTCSKCGHLNNYFNFEYRKKNKFPHFKCEKCNFKENADYNAALNISNPKLKSTKEEP

SEQ ID NO: 1544 - protein, 726 aa, synthetic construct
SEVEFSHEYWMRRALTLAKRARDEREVPVGAVLVLNNRVIGVGWNRAVGLHDPTAHAEIMALRQGGLVMQNYRLIEATLYVTFEPCIMCAGAMIHSRIGRVVFGVRNSKRGAAGSLMNVLNYPGMNHRVEITEGILADECAALLCDFYRMPRRVFNAQKKAQPSINSGGSSGGSSGSVTPGTSESATPESSGGSSGGSAKNTITKTLKLRIVRPYNSAEVEKIVADEKNNREKIALEKNKDKVKEACSKHLKVAAYCTTQVESNACLFCKARKLDDKFYQKLRGQFPDAVFWQEIGEIFRQLQKQAAEIYNQSLIELYYEIFIKGKGFANASSVEHYLSDVCYTRAAELFKNAAIASGLRGKVKSNFRLKELKNMKSGLPTTKSDNFPIPLVKQKGGQYTGFEISSHNDDFIVKIPFGRWQVKKEIDKYRPWEKFDFEQVRKNPKPISLLLSTQRRKRNKGWCKDESTEAEIKKVMNGDYQTSYIEVKRGSKVGEKSVWMLSLSIDVPKIDKGVDPSIIGGIDVGVKSPLVCAINNVLSRYSISDNDLFHFNKKMFARRRILLKKNGLKRAGHGAKNKLKPITIMTEKSKRFRKKLIERWACEIADFFIKNKVGTVQMENLESMKRKEDSYFNIRLRGFWPYAEMQNKIEFKLKQYGIEIRKVAPNNTSKTCSKCGHLNNYFNFEYRKMNKFPHFKCEKCNFKENADYNAALNISNPKLKSTKEEP

SEQ ID NO: 1545 - protein, 726 aa, synthetic construct
SEVEFSHEYWMRHALTLAKRARDEREVPVGAVLVLNNRAIGEGWNRAIGLHDPTAHAEIMALRQGGLVMQNYRLTDATLYVTFEPCVMCAGAMIHSRIGRVVFGVRNSKRGAAGSLMNVLNYPGMNHRVEVTEGILVDECAALLCDFYRMPRQVLNAQKKAQSSISSGGSSGGSSGSETPGASGSVTPKSSGGSSAGSTKDTITKTLKLRIVRPYNSAEVEKIVADEKNNREKIVMEKNKDKVKEACSKHLKVVSYCTTQVERNACLFCKARKLDDKFYQKLRGQFPDAVFWQELGGIFRQLQKQAAEIYNQSLIELYYEIFIKGKGFANASSAEHYLSDVCYTRAAELFKNAAIASGLRGKVKSNFRLKELKNMKSGLPTTKSDNFPIPLVKQKGGKYTGFEISSHNDDFIIKIPFGRWQVKKEIDKYRPWEKFDFEQVRKSPKPISLLLSTQRRKRNKGWSKDEGTEAEIRKVMNGDYQTSYIEVKRGRKIGEKSVWMLNLSIDVPKIDKGVDPSTIGGIDVGVKSPLVCAINNAFSRYSISDNDLFRFNKKMFARRRILLKKNRHKRAGHGAKNKLKPITILTEKSGRFRKKLIERWACEIADFFIKNKVGTVQMENLESMKRKEDSYFNIRLRGFWPYAEMQNKIELKLKQYGIKIRKVAPNNTSKTCSKCGHLNDYFNFEYRKKNKFPHFKCEKCNFKEDADYNAALNISNPKLKSTREEP

SEQ ID NO: 1546 - protein, 726 aa, synthetic construct
SEVEFSHEYWMRHALTLAKRARDEREVPVGAVLVLNNRVIGEGWNRAIGLHDPTAHAEIMALRQGGLVLQNYRLVDATLYVTFEPCVLCAGAMVHSRIGRVVFGARNSKRGAAGSLMNILNYPGMNHRVEITEGILADECAALLCDFYRMPRQVFNARKKAQSSINSGGSSGGSSGSETPGTSESATPESSGGSSGSSAKNTITKTLKLRIVRPYNSAEVEKIVADEKNNREKIALEKNKDKVKEACSEHLKVAAYCTTQVERSACLFCKARKLDDKFYQRLRGQFPDAVFWQEIGEIFRQLQKQAAEIYNQSLIELYYEIFIKGKGFANASSVEHYLSGVCYTRAAELFKNAAIASGLRGKVKSNFRLKELKNMRSGLPTTKSDNFPIPLVKQKGGQYTGFEISSHNDDFIIKIPFGRWQVKKEIDKYRPWEKFDFEQVRKSPKPISLLLSTQRRKRNRGWSRDEGTEAEIRKVMNGDYQTSYIEVKRGSKTGEKSAWMLNLSIDVPKIDKGVDPSIIGGIDVGVKSPLVCAINNAFSRYSISDNDLFRFNKKMFARRRILLKKNRHKRAGHGAKNKLKPISILTGKSERFRKKLIERWACEIADFFTKNKVGTVQMENLESMKGKEDSYFNIRLRGFWPYAEMQSKIEFKLKQYGIEVRKVAPNNTSKTCSKCGHLNNYFNFEFRKKNKFPHFKCEKCNFKEDADYNAALNISNPKLKSTKEEP

SEQ ID NO: 1547 - protein, 726 aa, synthetic construct
SEVEFSHEYWMRHALTLAKRARDEREVPVGAVLVLNNRVIGEGWNRAIGLHDPTAHAEIMALRQGGLVMQNYRLVDATLYVTFEPCVLCAGAMVHSRIGRVVFGVRNSKRGAAGSLMNVLNYPGMNHRVEVTEGILADECAALLCDFYRMPRQVFNAQKKARSNINSGGSSGGSSGSEMPGTSESATPESSGGSSGGSAKNTITKTLKLRIVRPYNSAEVEKIVADEKNNREKIALEKNKDKVKEACSKHLKVAAYCTTQVERNACLFCKARKLDDKFYQKLRGQFPDAVFWQEIGEIFRQLQKQAAEIYNQSLIELYYEIFIKGKGIANASSVEHYLSDVCYTRAAELFKNAAIASGLRNKVKSNFRLKELRSMKSGLPTTKSDNFPIPLVRQKGGQYTGFEISNHNSDFTIKIPFGRWQAKKEIDKYRPWEKFDFEQVRKSPKPISLLLSTQRRKRNKGWSRDEGTEAEIRKVMNGDYQTSYIEVKRGSKVGEKSAWMLSLSIDVPKIDKGVDPSIVGGIDVGVKSPLVCAINNALGRYSISDNDLFHFNKKMFARRRILLKKSKHKRAGHGAKNKLKPITILTEKSGRFRKKLIERWACEIADFFIKNKVGTVQMENLESMKRKEDSYFNIRLRGFWPYAEMQNKIEVKLKQYGIEIRKVAPNNTSKTCSKCGHLNSYFNFEYRKKNKFPHFKCEKCNFKENADYNAALNISNPKLKSTKEEP

SEQ ID NO: 1548 - protein, 726 aa, synthetic construct
SEVEFSHEYWMRRALTLAKRARDEREVPVGAILVLNNRVIGEGWNRAIGLHDPTAHAEIMALRQGGLVMQNYRLIDATLYVTFEPCVMCAGAMIHSRIGRVVFGVRNSKHGAAGSLMDVLNYPGMNHRVEITEGILADECAALLCDFYRMPRQVFNAQKKAQSSISSGGSSGGSNGSETPGTSESATPESSGGSSGGSAKNTITKTLKLKIVRPYNSAEVEKIVADEKNNREKIALEKNKDKVKEACSKHLKVAAYCTTQVERNACLFCRARKLDDKFYQRLRGQFPDAVFWQEIGEIFRQLQKQAAEIYNQSLIELYYEIFIKGKGFANASSVEHYLSDVCYTRAAELFKNAAIASGLRGKVKSNFRLKELKNMKSGLPTTKSDNFPIPLVKQKGGQYTGFEISNHNNDFIIKIPFGRWLAKKEIDKYRPWEKFDFEQVRKSPKPISLLLSTQRRKRNKGWSKDEGTEAEIRKVMNGGYQTSYIEVKRGSKTGEKSAWMLNLSIDVPKIDKGVDPSIIGGIDVGVKSPLVCAINNAFSRYSISDNDLFHFNKKMFARRRILLKKNRHKRTGHGAKNKLKPISILTEKSKRFRKKLIERWACEIADFFIKNKVGTVQMENLKSMKRREDSYFNIRLRGFWPYAEMQNKIEFKLKQYGIEIRKVAPNNTSKTCSKCGHLNNYFNFEYRRKNKFPHFKCEKCNFKEDADYNAALNISNPKLKSTKEEP

SEQ ID NO: 1549 - protein, 726 aa, synthetic construct
SEVEFSHEYWMRRALTLAKRARDEREVPVGAVLVLNNRVIGVGWNRAVGLHDPTAHAEIMALRQGGLVMQNYRLVEATLYVTFEPCIMCAGAMIHSRIGRVVFGVRNSKRGAAGSLMNVLYYPGMNHRVEITEGILADECAALLCDYYRMPRQVFNARKKAQSSINSGGSSDSGSGSETPGTSESATPESSGGSSGGSAKNTITKTLKLRIVRPYNSAEVEKIVADEKNNREKIALEKNKDKVKEACSEHLKVAAYCTTQVERSACLFCKARKLDDKFYQKLRGQFPDAVFWQEIGEIFRQLQKQAAEIYNQSLIELYYEIFIKGKGFANASSVEHYLSDVCYTRAAELFKNAAIASGLRGKVKSNFRLKELKNMKSGLPTTKSDNFPIPLVKQKGGQYTGFEISSHNGDFIIKIPFGRWQVKKEIDKYRPWEKFDFEQVRKSPKPISLLLSTQRRKRNKGWSKDEGTEAEIRKVMNGDYQTSYIEVKKGSKTGEKSAWMLNLSIDVPKIDKGVDPSIIGGIDVGVKSPLVCAINNAFSRYSISDNDLFHFNKKMFARRRILLKKNRHKRAGHGARNKLKPITVLTEKSERFRKKLIERWACEIADFFIKNKVGTVQMENLESMKRRGDSYFNIRLRGFWPYAEMQNKIEFKLKQYGVEIRKVAPNNTSKTCSKCGHLNYYFNFEYRKKNKFPHFKCEKCNFKEDADYNAALNISNPKLKSTKEEP

SEQ ID NO: 1550 - protein, 726 aa, synthetic construct
SEVEFSHEYWMRHALTLAKRARDEGEVPVGAVLVLNNRVIGEGWNRAIGLHDPTAHAEIMALRQGGLVMQNYRLVDATLYVTFEPCVLCAGAMVHSRIGRVVFGVRNSKRGAAGSLMNVLNYPGMNHRVEITEGILADECAALLCDFYRMPRQVFNARKKAQSSINPGGSSGGSSGSETPGTSESATPESSGGSSGSSAKNTITKTLKLRIVRPYNSAEVEKIVADEKNNREKIALEKNKDKVKEACSKHLKVAAYCTTQVERNACLFCKARRLDDKFYQKLRGQFPDAVFWQEIGEIFRQLQKQAAEIYNQSLIELYYEIFIKGKGIVNASSVEHYLSDVCYTRAAELFKNAAIASGLRSKVRSNFRLKELKNMKSGLPTTKSDNFPIPLVKQKGGQYTGFEISSHNSDFIIKIPFGRWQVKKEIDKYRPWEKFDFEQVRKSPKPISLLLSTQRRKRNKGWSKDEGTEAEIRKVMNGDYQTSYIEVKRGSKTGEKSAWMLNLSIDVPKIDKGVDPSIIGGIDVGVKSPLVCAINNAFSRYSISDNDLFRFNKKMFARRRILLKKNRHKRAGHGAKNKLKPISILTGKGERFRKKLIERWACEIADFFIKNKVGTVQMENLESMKRKEDSYFNIRLRGFWPYAEMQNKIEFKLKQYGIEIRKVAPNNTSKTCSKCGHLNNYFNFEYRKKNKFPHFKCEKCNFKENADYNAALNISNPKLKSTKEEP

SEQ ID NO: 1551 - protein, 726 aa, synthetic construct
SEVEFSHEYWMRHALTLAKRARDEREVPVGAVLVLNNRVIGEGWNRAIGLHDPTAHAEIMALRQGGLVMQNYRLADATLYVTFEPCVMCAGAMIHSRIGRVVFGVRNSKRGAAGSLMNVLNYPGMNHCVEITESILVDECAALLCDFYRMPRQVLNAQKKAQSSISSGGSSGGSSGSETPGASGSVTPKSSGGSSAGSAKDTITKTLKLRIVRPYNSAEVEKIVADEKNSREKIALEKNKDKVKEACSKHLKVAAYCTTQVERNACLFCKARKLDDKFYQKLRGQFPDAVFWQEIGEIFRQLQKQAAEIYNQSLIELYYEIFIKGKGLANASSVEHYLSDVCYTRAAELFKNAAIASGLRGKVKSNFKLKELKSMKSGLPSTKSDNFPIPLVKQKGGQYTGFEIRGHNDDLIIKIPFGRWQVKEEIDKYRPWEKFDFEQVRKSPKPISLLLSTQRRRRNKGWSKDEGTEAEIRKVMNGDYQTSYIEVKRGSKIGEKSAWMLNLSIDVPKIDKGVDPSIIGGIDVGVKSPLVCAINNAFSRYSISDNDLFHFNKKMFARRRILLKKNRHKRAGHGAKNKLKPISILTEKSKRFRKKLIERWACEIADFFIKNKVGTVQMENLESMKRKEDSYFNIRLRGFWPYAEMQNKIEFKLKQYGIEIRKVAPNNTSKTCSKCGHLNNYFNFEYRKMNKFPHFKCEKCNFKENADYNAALNISNPKLKSTKEEP

SEQ ID NO: 1552 - protein, 726 aa, synthetic construct
SEVEFSHEYWMRHALTLAKRARDEREVPVGAILVLNNRVIGVGWNRAIGLHDPTAHAEIMALRQGGLVMQNYRLVDATLYVTFEPCVMCAGAMIHSRIGRVVFGVRNSKHGAAGSLVNVLNYPGMNHRVEITEGILADECAALLCDFYRMPRQVFNAQKKAQSSINSGGSSGGSSGSETPSTSESATPESSGGSSGGSAKNTITKTLQLRIVRPYNSAEVEKIVTDEKNNREKIALEKNKDKVKEACSKHLKMASYCTTQVERNACLFCKARKLDDKFYQKLRGQFPNAVFWQELGGIFRQLQKQAAEIYNQSLIELYYEIFIKGKGITNASRVEHYLSDVCYTRAAELFKNAAIASGLRSKVRSNFRLKELKNMKSGLPTTKSDNFPIPLVKQKGGQYTGFEISSHNSDFIIKIPFGRWQVKEEIDKFRPWEKFDFEQVRKSPKPISLLLSTQRRKKNKGWSKDEGTEAEIRKVMNGDYQTSYIEVRRGSKIGEKNAWMLNLSIDVPKIDKGVDPSIIGGIDVGVKSPLVCAINNAFSRYSISDNDLFRFNKKMFARRRILLKKNRHKRAGHGAKNKLKPISILTGRSERFRKKLIERWACEIADFFIKNKVGTVQMENLESMKRREDSYFNIRLRGFWPYAEMQSKIEFKLKQYGIEIRKVAPNNTSKTCSKCGHLNNYFNFEYRKKSKFPHFKCEKCNFKENADYNAALNISNPKLKSTKEEP

SEQ ID NO: 1553 - protein, 726 aa, synthetic construct
SEVEFSHEYWMRHALTLAKRARDEREVPVGAVLVLNNRVIGEGWNRAIGLHDPTAHAEIMALRQGGLVMQNYRLIDATLYVTFEPCVMCAGAMIHSRIGRVVFGVRNSKRGAAGSLMNVLNYPGMNHCVEITEGILADECAALLCDFYRMPRQVLNAQKKAQSSISPGGSSGGSSCCETPGASESVTPKSSGGSSAGSTKNTITKTLKLRIVRPYNSAEVEKIVADEKNSREKIALEKNKDKVREACSEHLKVAAYCTTQVERNACLFCKARKLDDKFYQKLRGQFPDAVFWQEIGEIFRQLQKQAAEIYNQSLIELYYEIFIKGKGIANASSVGHYLSNVCYTRAAELFKNAAIASGLRGKIKSNFRLKELKNMKSGLPTTKSDNFPIPLVKQKGGQYTGFEISSHDDDFVIKIPFGRWQVKKEIDKYRPWEKFDFEQVRKGPKPISLLLSTQRRKRNKGWSKDEGTEAEIRKVMNGDYQTSYIEVKRGSKIGEKSAWMLNLSIDVPKIDKGVDPSIIGGIDVGVKSPLVCAINNALSRYSISDNDLFHFNKKMFARRRILLRKNRHKRAGHGARNKLKPITVLTEKSERFRKKLIERWACEIANFFIKNKVGTVQMENLESMKRREDSYFNIRLRGFWPYAEMQNKIEFKLKQYGIVVRKVAPNNTSKTCSKCGHLNHYFNFEYRKKNKFPHFKCEKCNFKEDADYNAALNISNPKLKSTKGEP

SEQ ID NO: 1554 - protein, 726 aa, synthetic construct
SEVEFSHEYWMHHALTLAKRARDEREVPVGAILVLNNRVIGEGWNRAIGLHDPTAHAEIMALRQGGLVMQNYRLIDATLYVTFEPCVMCAGAMIHSRIGRVVFGVRNSKHGAAGSLVNVLNYPGMNHRVEITEGILADECAALLCDFYRMPRQVFNARKKAQSSINSGGSSGDSSGSETPGTSESATPKSSGGSSGGSAKNTITKALKLRIVRPYNSAEVEKIVADEKNNRERIALEKNKDKVKEACSKHLKVAAYCTTQVERNACLFCKARKLDDKFYQKLRGQFPDAVFWQEIGEIFRQLQKQAAEIYNQSLIELYYEIFIKGKGFANASSVEHYLSDVCYTRAAELFKNAAIASGLRGKVKSNFRLKELKNMRSGLPTTKSDNFPIPLVKQKGGQYAGFEISSHNDDFIIKIPFGRWQVKKEIDRYRPWEKFDFEQVRKSPKPISLLLSTQRRKRNKGWSKDEGTEAEIRKVMNGDYQTSYIEVKRGSKTGEKSAWMLNLSIDVPKIDKGVDPSIIGGIDVGVKSPLVCAINNAFSRYSISDNDLFRFNKKMFARRRILLKKNRHKRAGHGAKNKLKPISILTGKSERFRKKLIERWACEIADFFIKNKVGTVQMENLESMKRREDSYFNIRLRGFWPYAEMQNKIEFKLKQYGIEIRKVAPNNTSKTCSKCGHLNNYFNFEYRKKNKFPHFKCEKCNFKENADYNAALNISNPKLKSTKEEP

SEQ ID NO: 1555 - protein, 726 aa, synthetic construct
SEVEFSHEYWMRHALTLAKRARDEREVPVGAILVLDNRVIGVGWNRAIGLHDPTAHAEIMALRQGGLVMQNYRLIDATLYVTFEPCVMCAGAMIHSRIGRVVFGVRNSKHGAAGSLVNVLNYPGMNHRIEITEGILADECAALLCDFYRMPRQVFNARKKAQSSINSGGSSGGSSGSETPGTSESATPKNSGGSSGGSAKNTITKALKLKIVRPYNSAEVEKIVADEKNNRERIALEKNKDKVKEACSKHLKVAAYCTTQVERNACLFCKARKLDDKFYQKLRGQFPDAVFWQEIGEIFRQLQKQAAEIYNQSLIELYYEIFIKGKGFANASSVEHYLSDVCYTRAAELFKNAAIASGLRGKVKSNFRLKELKNMRSGLPTTKSDNFPIPLVKQKGGQYAGFEISSHNGDFIIKIPFGRWQVKKEIDKYRPWEKFDFEQVRKSPKPISLLLSTRRRKRNKGWSKDEGTEAEIRKVMNGDYQTSYIEVKRGSKIGEKSAWMLNLSIDVPKIDKGVDPSIIGGIDVGVKSPLVCAINNAFGRYSISDNDLFHFNKKMFARRRILLKKNRHKRAGHGAKNKLKPITILTEKSKRFRKKLIERWACEIADFFIKNKVGTVQMENLESMKRKEDSYFNIRLRGFWPYAEMQDKIEFKLKQYGIEIRKVAPNNTSKTCSRCGHLNNYFDFEYRRKNKFPHFKCEKCNFKENADYNAALNISNPKLKSTKEEP

SEQ ID NO: 1556 - protein, 726 aa, synthetic construct
SEVEFSHEYWMRHALTLARRARDEREVPVGAILVLNNRVIGEGWNRAIGLHDPTAHAEIMALRQGGLVMQNYRLVDATLYVTFEPCVMCAGAMIHSRIGRVVFGVRNNKHGAAGSLMNVLNYPGMNHRVEITEGILADECAALLCDFYRMPRQVFNARKKAQSSINPGGPSGGSSGSKTPGTSESATPEGSGGSSGGSAKNTITKTLKLRIVRPYNSAEVEKIVADEKNNREKIALEKNKDKVKEACSKHLKVAAYCTTQVERNACLFCKARRLDDKFYQKLRGQFPDAVFWQEIGEIFRQLQKQAAEIYNQSLIELYYEIFIKGKGTANASSVEHYLSDVCYTRAAELFKNAAIASGLRGKVKSNFRLKELKNMRSGLPTTKSDNFPIPLVKQKGGQYTGFEISNHNDDFIIKIPFGRWQVKKEINKFRPWEKFDFEQVRKSPKPLSLLLSTQRRKRNKGWSTDEGTEAEIRKVMNGGYQTSYIEVKRGSKVGEKSAWMVNLSIDVPKIDKGVDPSIIGGIDVGVKSPLVCAVNNALSRYSIDDNDLFHFNKKMFARRRILLKKSRHKRAGHGAKNKLKPITILTEKSRRFRKKLIERWACEIADFFIKNKVGTVQMENLESMKRKEDSYFNIRLRGFWPYAEMQNKIEFKLKQYGIEIRKVAPNNTSRTCSKCGHLNNYFNFEYRKKNKFPHFKCERCSFKENADYNAALNISNPKLKSTKEEP

SEQ ID NO: 1557 - protein, 726 aa, synthetic construct
SEVEFSHEYWMRHALTLAKRARDEREVPVGAILVLNNRVIGEGWNRAIGLHDPTAHAEIMALRQGGLVMQNYRLIDATLYVTFEPCVMCAGAMIHSRIGRVVFGVRNNKHGAAGSLVNVLNYPGMNHRVEITEGILADECAALLCDFYRMPRQVFNARKKAQSSISSGGSSGGSSGSETPGASESVTPKGSVGSSAGPTKNTITKTLKLRIVRPYNSAEVEKIVADEKNNRERIALEKNKDKVKEACSKHLKVATYCTTQVERNACLFCKARRLDDKFYQKLRGQFPDAVFWQEIGEIFRQLQKQAAEIYNQSLVELYYEILIKGKGIANASSVEHYLSDVCYTRAAELFKNAAIASGLRGKVKSNFRLKELKNMKSGLPTTKSDNFPIPLVKQKGGQYTGFEISSHNDDFIIKIPFGRWQVKKEIDKYRPWEKFDFEQVRKNPKPISLLLSTLRRKRNKGWSKDEGTEAEIRKVMNGDYQTSYIEVKRGSKVGEKSAWMLNLSIDVPKIDKGADPSIIGGIDVGVKSPLVCAINNALSRYSISDNDLFHFNKKVFARRRILLRKNRHKRAGHGAKNKLKPITILTEKSERFRKKLIERWACEIADFFIKNKVGTVQMENLESMKRKEDSYFNIRLRGFWPYAEMQSKIEFKLKQYGIVVRKVAPNNTSKTCSQCGHLNNYFNFEYRKKNKFPYFKCEKCNFKENADYNAALNISNPQLKSTKGEP

SEQ ID NO: 1558 - protein, 726 aa, synthetic construct
SEVEFSHEYWMRHALTLARRARDEGEVPVGAVLVLNNRVIGEGWNRAIGLHDPTAHAEIMALRQGGLVMQNYRLVDATLYVTFEPCVLCAGAMVHSRIGRVVFGVRNSKRGAAGSLMNVLNYPGMNHRVEITEGILADECAALLCDFYRVPRQVFNAQKKARSDINSGSSSGGSSGSETPGTSESATPESSGGSSGGSAKNTITKTLQLRIVRPYNSAEVEKIVADEKNNREKIALEKNKDKVKEACSKHLKVAAYCTTQVERNACLFCKARKLDDKFYQKLRGQFPDAVFWQEIGEIFRQLQKQAAEIYNQSLIELYYEIFIKGKGFAIASSVEHYLSCVCYTRAAELFKNAAIASGLRGKVKSNFRLKELKNMKSGLPTTKSDNFPIPLVKQKGGQYTGFEISSHDDDFIIKIPFGRWQVKKEIDKYRPWEKFDFEQVRKSPKPISLLLSTQRRKRSKGWSKDEGTEAEIRKVMNGDYQTSYIEVKRGSKTGEKSAWMLNLSIDVPKIDKGVDPSIIGGIDVGVKSPLVCAINNAFSRYSISDNDLFRFNKKVFARRRILLKKNRHKRAGHGTKNKLKPITILTEKSARFRKKLIERWACEIADFFIRNKVGTVQMENLESMKRKEDSYFNIRLRGFWPYAEMQNKIEFKLKQYGIKIRKVAPNNTSKTCSKCGHLNNYFGFEYRKKNKFPHFKCEKCNFKEDADYNAALNICNPKLKSTKEEP

SEQ ID NO: 1559 - protein, 725 aa, synthetic construct
SEVEFSHEYWMRHALTLAKRARDEREVPVGAILVLNNRVIGEGWNRAIGLHDPTAHAEIMALRQGGLVMQNYRLIDATLYVTFEPCVMCAGAMIHSRIGRVVFGVRNNKHGAAGSLVNVLNYPGMNHRVEITEGILADECAALLCDFYRMPRQVFNARKKARSNINSGGSSGGSSGSETPGTSKSATPESSGGSSGGSTKNTITKTLKLRIVRPYNSAEVEKIVADEKNNREIALEKNKDKVKEACSKHLKVAAYCTTQVERNACLFCRARRLDDKFYQKLRGQFPDAVFWQEIGEVFRQLQKQAAEIYNQSLVELYYEIFIKGKGIANTSSVEHYLSDVCYTRAAELFKNAAIASGLRGKVKSNFRLKELKNMRSGLPTTKSDNFPIPLVKQKGGQYAGFEISSHNDDFIIKIPFGRWQVKKEIDKYRPWEKFDFEQVRKSPKPISLLLSTRRRKGNKGWSKDEGTEAEIRKVMNGDYQTSYIEVKRGSKIGEKSAWMLNLSIDVPKIDKGVDPSIIGGIDVGVKSPLVCAINNAFSRYSISDNDLFHFNKKVFARRRILLKKNRHRRAGHGAKNKLKPITILTEKSKRFRKKLIERWACEIADFFIKNKVGTVQMENLESMKRKEDSYFNIRLRGFWPYAEMQNKIEFKLKQYGIKIRKVAPNNTSRTCSECGHLNNYFSFEYRKKNKFPHFKCEKCNFKEDADYNAALNISNPKLKSTKEEP

SEQ ID NO: 1560 - protein, 726 aa, synthetic construct
SEVEFSHEYWMRHALTLAKRARDEREVPVGAILVLNNRVIGEGWNRAIGLHDPTAHAEIMALRQGGLVMQNYRLTDATLYATFEPCVMCAGAMIHSRIGRVVFGVRNSKHGAAGSLMNVLNYPGMNHRVEITEGILADECAGLLCDFYRMPRQVFSARKKAQSSINPGGSTSGSSGGKAPGTSESATLESSGGSSGDSAKNSITKTLKLRIVRPYNSAEVEKIVADEKNNREKIALERNKGKVKEACSKHLKVASYCTTQVERNACLFCKARKLDDKFYQELRGQFPDAVFWQEIGEIFRQLQKQAAEIYNQSLIELYYEIFIKGKGIVNASSVGHYLSDVCYTRAAELFKNAAIASGLRSKIKSNFRLKELRNMRGGLPTTKSDNFPIPLVKQKGGQYTGFEISSHNDDFIIKIPFGRWQVKKEIDKYRPWEKFDFEQVRKSPKPISLLLSTQRRKRNKGWSKDEGTEAEIRKVMNGDYQTSYIEVKRGSKIGEKSAWMLNLSIDVPKIDKGVDPSIVGGIDVGVKSPLVCAIDNALSRYSISDNDLFHFNKKMFARRRILLKKNRHRRAGHGAKNKLKPISILTEKSKRFRKKLIERWACEIADFFIKNKVGTVQMENLESMKRKEDSYFNIRLRGFWPYAEMQNKIEFKLKQYGIEIRKVAPNNTSKTCSKCGHLNNYFNFEYRKKNKFPHFKCEKCNFKEDADYNAALNISNPKLKSTKEEP

SEQ ID NO: 1561 - protein, 726 aa, synthetic construct
SEVEFSHEYWMRHALTLAKRARDEREVPVGAVLVLNNRVIGEGWNRAIGLHDPTAHAEIMALRQGGLVTQNYRLIDATLYVTFEPCVMCAGAMIHSRIGRVVFGVRNSKRGAAGSLMNVLNYPGMDHRVEITEGILADECAALLCDFYRMPRQVFNARRKAQSSITSGGSSGGSSGSETPGTSESATPESSGGSSGGSAKNTITKTLKLRIVRPYNSAEVERILADEKDNREKIALERNKDKVKEACSKHLKVAAYCTTQVERNACLFCRARKLDDKFYQKLRGQFPDAVFWQEIGEIFRQLQKQAAEIYNQSLIELYYEIFIKGKGITNASRVEHYLSDVCYTRAAELFKNAAIASGLRGKVKSNFRLKELKSMKSGLPTTKSDNFPIPLVKQKGGQYTGFEISSHNSDFIIKIPFGRWQVKEEIDKYRPWEKFDFEQVRKSPKPISLLLSTQRRKKNKGWGKDEGTEAEIRKVMNGDYQTSYIEVKRGSKIGEKSAWMLNLSIDVPKIDKGVDPSIVGGIDVGVKSPLVCAIDNALSRYSISDNDLFHFNKKMFARRRILLKKNRHRRAGHGAKNKLKPISILTGKSKRFRKKLIERWACEIADFFIKNKVGTVQMENLESMKRKEDSYFNIRLRGFWPYAEMQNKIEFKLKQYGIEIRKVAPNNTSKTCSKCGHLNNYFNFEYRKKNKFPHFKCEKCNFKENADYNAALNISNPKLKSTKGEP

SEQ ID NO: 1562 - protein, 726 aa, synthetic construct
SEDEFSHEYWMRHALTLAKRARDGREVPVGAVLVLNNRVIGEGWNRAIGLHDPTAHAEIMALRQGGLVMQNYRLIDATLYVTFEPCVMCAGAMIHSRIGRVVFGVRNSKRGAAGSLMNVLNYPGMNHRVEITEGILAGECAALLCDFYRMPRQVFNAQKKAQSTINSGGSSGGSSSSETPGTSGSATPEGSGGSSGGSAKNTITKTLKLRIVRPYNSAEVEKIVADEKNNREKIALEKNKDKVKEACSKHLKVASYCTTQVERNACLFCKARKLDDRFYQKLRGQFPDAVFWQEIGEIFRQLQKQAAEIYNQSLIELYYEIFIKGKGFANASSVEHYLSDVCYTRAAELFKNAAIASGLRGKVKSNFRLKELKNMKSGLPTTKSDNFPIPLVRQKGGQYTGFEVSSHNDDFIIKIPFGRWQVKKEIDKYRPWEKFDFEQVRKSPRPISLLLSTQRRKRNKGWSKDEGTEAEIRKVMNGDYQTSYIEVKRGSKVGEKSAWMLNLSIDVPKVDKGVDPSIIGGIDVGVKSPLVCAINNAFSRYSISDNDLFRFNKKVFARRRILLKKNRHRRAGHGAKNKLKPITILTEKSKRFRKKLIERWACEIADFFIKNKVGTVQMENLESMKRKEDSYFNIRLRGFWPYAEMQNKIEFKLKQYGIKIRKVAPNNTSRTCSKCGHLNNYFSFEYRKKNKFPHFKCEKCNFKEDADYNAALNISNPKLKGTKEEL

SEQ ID NO: 1563 - protein, 726 aa, synthetic construct
SEVEFSHEYWMRHALSLAKRARDEREVPVGAVLVLNNRIIGEGWNRAIGQHDPTAHAEIMALRQGGLVMQNNRLTDATLYVTFEPCVMCAGAMVHSRIGRVVFGVRNSKRGAAGSLMNVLNYPGVNHCVEITEGILVDECAALLCDFYRMPRQVLNAQKRTQSSINSGGSSGGSSGSETPGTSESATPESSGGGSSGSAKNTITKTLQLRIVRPYNSAEVEKIVADEKNNREKIALEKNKGRVKEACSKHLKVASYCTTQVERNACPFCKARKLDDKFYQKLRGQFPDAVFWQELGEILRQLQKQAAEIYNQSLIELYYEIFIKGRGFANASSVEHYLSDVCYTRAAELFKNAAIASGLRGKVKSNFRLKELKNMKSGLPTTKSDNFPIPLVKQKGGQYTGFEISSHNDDFIIKIPFGRWQVKKEIDKYRPWEKFDFEQVRKSPRPISLLLSTQRRKRNKGWSKDEGTEAEIRKVMNGDYRTSYIEVKRGSKVGEKSAWMLNLSIDVPKIDKGVDPSIIGGIDVGVKSPLVCAINNAFSRYSISDNDLFHFNKKMFARRRILLKKNRHRRAGHGAKNKLKPIAVLAEKSEGFRKKLIERWACEVADFFIKNKVGTVQMENLESMKRREDSYFNIRLRGFWPYAEMQNKIEFKLKQYGIKIRKVAPNNTSKTCSKCGHLNNYFSFEYRKENKFPHFKCEKCNFKENADYNAALNISNPKLMSTKEEP

SEQ ID NO: 1564 - protein, 726 aa, synthetic construct
SEVEFSHEYWMRHALTLAKRARDEREVPVGAVLVLNNRVIGEGWNRTTGLHDPTAHAEIMALRQGGLVMQNHRLVDATLYVTFEPCVLCAGAMVHSRIGRVVFGVRNSKRGAAGSLMNVLNHPGMNHRVEITGGILADECAALLCDFYRMPRQVFNAQKKARSNINSGGSSGGSSGSETLGTSESATPESSGGSSGGSAKNTIAKTLKLRIVRPYNSAEVEKIVADEKNNREKIALEKNKDKVKEACSKHLKVAAYCTTQVERNACLFCKARKLDDKFYQKLRGQFPDAVFWQEIGEIFRQLQKQAAEIYNQSLIELYYEIFIKGKGFANASSVEHYLSDVCYTRAAELFKNAAIASGLRGKVKSNFRLKELKNMKSGLPTTKSDNFPIPLVKQKGGQYTGFEISSHNDDFIIKIPFGRWQVKKEVDKYRPWEKFDFEQVRKSPKPISLLLSTQRRKRNKGWGKDEGTEAEIRKVMNGDYQTSYIEVKRGSKIGEKSAWMLNLSVDVPKIDKGVDPSIIGGIDVGVKSPLVCAINNALSRYSISDNDLFHFNKRMFARRRILLRGNRHKRAGHGAKNKLKPITILTEKSKRFRKKLIERWACEIADFFIKNKVGTVQMENLESMKRKEDSYFNIRLRGFWPYAEMQNKIEFKLKQYGIKIRKVAPNNTSKTCSKCGHLNNYFNFEYRKRNKFPHFKCEKCNFKENADYNAALNISNPKLKGTKEEP

SEQ ID NO: 1565 - protein, 726 aa, synthetic construct
SEDEFSHEYWMRHALTLAKRARDGREVPVGAVLVLNNRVIGEGWNRAIGLHDPTAHAEIMALRQGGLVMQNYRLIDATLYVTFEPCVMCAGAMVHSRIGRVVFGVRNSKRGAAGSLMNVLDYPGMGHRVEITEGILADECAALLCDFYCMPRQVFNAQKRAQSCINSGGSSGGSSGSETPSTSESATPGSSGGGSSGSAKNTITKTLQLRIVRPYNSAEVEKIVADEKNNREKIALEKNKDKVKEACSKHLKVASYCTTQVERNACPFCKARKLDDKFYQKLRGQFPDAVFWQELGEILRQLQKQAAEIYNQSLIELYYEIFIKGKGFANASSVEHYLSDVCYTRAAELFKNAAIASGLRGKVKSNFRLKELKNMKSGLPTTKSDNFPIPLVKQKGGQYTGFEISSRNDDFIIKIPFGRWQVKKEIDKYRPWEKFDFEQVRKSPKPISLLLSTQRRKRNKGWSKDEGTEAEIRKVMNGDYQTSYIEVKRGSKIGEKSAWMLNLSIDVPKIDKGVDPSIIGGIDVGVKSPLVCAINNAFSRYSISDNDLFHFNKKMFARRRILLKKNRHKRAGHGAKNKLKPISILTEKSGRFRKKLIERWACEIADFFIKNKVGTVQMENLESMKRKEDSYFNIRLRGFWPYAEMQNKIEFKLKQCGIKIRKVAPNNTSKTCSKCGHLNNYFSFEYRKKNKFPHFKCEKCNFKENADYNAALNISNPKLKSTKEEP

SEQ ID NO: 1566 - protein, 726 aa, synthetic construct
SEVEFSHEYWMRHALTLAKRARDEREVPVGAILVLNNRVIGEGWNRAIGLHDPTAHAEIMALRQGGLVMQNYRLVNATLYVTFEPCVMCAGAMIHSRIGRVVFGARNSKRGAAGSLMNVLNYPGMNHRVEITEGILTDECAALLCDFYRMPHQVLNAQKKAQSSINSGGSSDGSSGSVTPGTSGSATPEGSGGSSAGSTKNTITKTLKLRIVRPYNSAEVEKIVADEKNSREKIALERNKDKVKEACSEHLKVAAYCTTQVERNACLFCKARKLDDRFYQKLRGQFPDAVFWQETGEIFRQLQRQAAEIYNQSLIELYYEIFIKGKGFANASSVEHYLSDVCYTRAAELFKNAAIASGLRGKVKSNFRLKELKNMKSGLPTTKSDNFPIPLVKQKGGQYTGFEISSHNDDFIIKIPFGRWQVKKEIDRYRPWEKFDFAQVRKSPKPISLLLSTQRRKRNRGWSKDEGTEAEIKKVMNGDYQTSYIEVKRGSKIGEKSAWMLNLSIDVPKIDKGVDPSIIGGIDVGVKSPLVCAINDAFSRYSISDNDLFHFNKKMFARRRILLKKSKHKRAGHGAKNKLKPITIMTEKSKRFRKKLIERWACEIADFFIKNKVGTVQMENLESMKRKEDSYFNIRLRGFWPYAEMQNKIEFKLKQYGIKIRKVAPNNTSKTCSKCGHLNNYFNFEYRKKNKFPHFKCEKCNFKEDADYNAALNISNPKQKSTKEEP

SEQ ID NO: 1567 - protein, 726 aa, synthetic construct
SEVEFSHEYWMRHALTLAKRARDEREVPVGAILVLNNRVIGEGWNRAIGLHDPTAHAEIMALRQGGLVMQNYRLTDATLYATFEPCVMCAGAMIHSRIGRVVFGVRNSKHGAAGSLMNVLNYPGMNHRVEITEGILADECAGLLCDFYRMPRQVFSARKKAQSSINPGGSSGGSSGGKAPGTSESATLESSGGSSSGSAKNSITKTLKLRIVRPYNSAEVEKIVADEKNNREKIALEKNKGKVEEACSKHLKVAAYCTTQVERNACLFCKARKLDDRFYQKLRGQFPDAVFWQEIGEIFRQLQKQAAEIYNQSLIELYYEIFIEGKGSANARSVEHYLSDVCYTRAAELFKNAAIASGLRGKVKGNFRLKELKSMKSGLPTTKSDNFPIPLVKQKGGQYTGFEISSHNDDFIIKIPFGRWQVKKEIDKYRPWEKFDFEQVRKSPKPISLLLSTQRRKRNKGWSKDEGTEAEIRKVMNGDYQTSYIEVKRGSKIGEKSAWMLNLSIDVPKIDKGVDPSIIGGIDVGVKSPLVCAINNAFSRYSISDNDLFHFNKKVFARRRILLKKNRHRRAGHGAKNKLKPITILTEKSKRFRKKLIERWACEIADFFIKNKVGTVQMENLESMKRKEDSYFNIRLRGFWPYAEMQNKIEFKLKQYGIKIRKVAPNNTSRTCSKCGHLNNYFSFEYRKKNKFPHFKCEKCNFKEDADYNAALNISNPKLKGTKEEP

SEQ ID NO: 1568 - protein, 726 aa, synthetic construct
SEDEFSHEYWMRHALTLAKRARDGREVPVGAVLVLNNRVIGEGWNRAIGLHDPTAHAEIMALRQGGLVMQNYRLIDATLYVTFEPCVMCAGAMVHSRIGRVVFGVRNSKRGAAGSLMNVLDYPGMGHRVEITEGILADECAALLCDFYRMPRQVFNARKKAQSSINPGGSSGGSGGSETPGTSESTTPEGSGSSSGGSAKNTITKTLKLRIVRPYNSAEVEKIVADEKNNREKIALEKNRDKVKEACSKHLKVASYCTTQVERNACPFCKARKLDDKFYQKLRGQFPDAVFWQELGEILRQLQKQAAEIYNQSLIELYYEIFIKGRGFANASSVEHYLSDVCYTRAAELFKNAAIASGLRGKVKSNFRLKELKNMKSGLPTTKSDNFPIPLVKQKGGQYTGFEISSHNDDFIIKIPFGRWQVKKEIDKYRPWEKFDFEQVRKSPKPISLLLSTQRRKRNKGWSKDEGTEAEIRKVMNGDYQTSYIEVKRGSKTGEKSAWMLNLSIDVPKIDKGVDPSIIGGIDVGVKSPLVCAINNAFCRYSISDNDLFHFNKKMFARRRILLKKSRHKRAGHGAKNKLKPISILTEKSKRFRKKLIERWACEIADFFIKNKVGTVQMENLESMKRKEDSYFNIRLRGFWPYAEMQNKIEFKLKQYGIEIRKVAPNNTSKTCSKCGHLNNYFNFEYRKKNKFPHFKCEKCNFKENADYNAALNISNPKLKSTKEGP

SEQ ID NO: 1569 - protein, 726 aa, synthetic construct
SEVEFSHEYWMRHALTLAKRARDEREVPVGAVLVLNNRVIGEGWNRAIGLHDPTAHAEIMALRQGGLVMQNHRLTDATLYVTFEPCVMCAGAMIHSRIGRVVFGVRNSKHGAAGSLVNVLNYPGMNHRVEITEGILADECAALLCDFYRMPRQVFGARRKAQSSINPGGSSGGSSVSETPGTSESPTPESPGGSSGGSAKNTITKTLKLRIVRPYNSAEVEKFVADEKNHREKIALEKNKDKVKEACSKHLKVAAYCTTQVERNACLFCKARKLDDKFYQKLRGQFPDAVFWQELGEILRQLQKQAAEIYNQSLIELYYEIFIKGRGFANASSVEHYLSDVCYTRAAELFKNAAIASGLRGKVKSNFRLKELKNMKSGLPTTKSDNFPIPLVKQKGGQYTGFEISSHNDDFIIKIPFGRWQVKKEINKYRPWEKFDFEQVRKSPKPISLLLSTQRRKRNKSWSKDEGTEAEIRKVMNGDYQTSYIEVKRGSKIGEKSAWMLSLSIDVPKIDKGVDPSIIGGIDVGVKSPLVCAINNALSRYSISDNDLFHFNKKVFARRRILLKKNRHRRAGHGARNKLKPITVLTEKSERFRKKLIERWACEIANFFIKNKVGTVQMENLESMKRREDSYFNIRLRGFWPYAEMQSKIEFKLKQYGIKIRKVAPNNTSKTCSKCGHLNNYFNFEFRKKNKFPHFKCEKCNFKEDADYNAALNISNPKLKGTKEEP

SEQ ID NO: 1570 - protein, 726 aa, synthetic construct
SEVEFSHEYWMRHALTLAKRARDEREVPVGAILVLNNRVIGEGWNRAIGLHDPTAHAEIMALRQGGLVMQNYRLIDATLYVTFEPCVMCAGAMIHSRIGRVVFGVRNNKHGAAGSLVNVLNYPGMNHRVEITEGILADECAALLCDFYRMPRQVFNARKKAQSSINPGGSSGGSSGSETPGTSESATPESSGGSSGGSAKNTITKTLTLRIVRPYNSAEVEKIVADEKNNREKIALEKNKDKVKEACSEHLKVATYCTTRVERNACLFCKARKLDDKFYQKLRGQFPDAVFWQELGEIFRQLQKQAAEIYNQSLIELYYEIFIKGKGFANASSVEHYLSDVCYTRAAELFKNAAIASGLRGKVKSNFRLKELRNMKSGLPTTKSDNFPIPLVRQKGGQYTGFEISSHNDDFIIKIPFGRWQVKKEIDKYRPWEKFDFEQVRKSPKPISLLLSTQRRKRNKGWSKDEGTEAEIRKVMNGDYQTSYIEVKRGSKTGEKSAWMLNLSIDVPKIDKGVDPSVIGGIDVGVKSPLVCAINNAFSRYSISDNDLFRYNKKMFARRRILLKKNRHKRAGHGARNKLKPISILTEKSKRFRKKLIERWACEIADFFIKNKVGTVQIENLESMKRREDSYFNIRLRGFWPYAEMQNKIEFKLKQYGIEIRKVAPNNTSKTCSKCGHLNSYFNFEYRKKNKFPHFKCEKCNFRENADYNAALNISNPKLRSTKEEP

SEQ ID NO: 1571 - protein, 726 aa, synthetic construct
SEVEFSHEYWMRHALTLAKRARDEREVPVGAVLVLNNRVIGEGWNRAIGLHDPTAHAEIMALRQGGLVMQNYRLTDATLYVTFEPCVMCAGAMIHSRIGRVVFGVRNSKRGAAGSLMNVLNYPGMNHCVEITEGILVDECAALLCDFYCMPRQVFNAQKRAQSSINSGGSSGGSSGSETPGASGSVTPKSSVGSSAGSTRNTITKTLKLRIVRPYNSAEVERIVADEKNNREKIALEKNKDKVKEACSKHLKVAAYCTTQVERNACLFCKARKLDDKFYQKLRGQFPDAVFWQELGEIFRQLQRQAAEVYNQSLIELYYEIFVKGKGFANASSVEHYLSDVCYTRAAELFKNAAIASGLRGKVKSNFRLKELRSMRSGLPTTKSDNFPIPLVKQKGGQYTGFEISSHNDDFIIKIPFGRWQVKKEIDKYRPWEKFDFEQVRKSPNPISLLLSTQRRKRNKGWSKDEGTEAEIRKVMNGDYQTSYIEVKRGSKVGEKSAWMLNLSIDVPKIDKGVDPSIIGGIDVGVKSPLVCAINNAFSRYSISDNDLFRFNKKVFARRRILLKKNRHKRAGHGTKNKLKPITILTEKSGRFRKKLIERWACEIANFFIKNKVGTVQMENLESMKRKEDSYFNIRLRGFWPYAEMQNKIEFKLKQYGIEIRKVAPHNTSRTCSKCGHLNNYFNFEYRRKNKFPHFKCEKCNFKEDADYNAALNISNPKLKSTMEEP

SEQ ID NO: 1572 - protein, 726 aa, synthetic construct
SEVEFSHEYWMRHALTLAKRARDEREVPVGAVLVLNNRVIGEGWNRAIGLHDPTAHAEIMALRQGGLVLQNYRLVDATLYVTFEPCVLCAGAMVHSRIGRVVFGARNSKRGAAGSLMNILNYPGMNHRVEITEGILADECAALLCDFYRMPRQVFNAQKKAQSSINSGGSSGGSSGGETPSTSESATPESSGGSSGGSAKNTITKTLQLRIVRPYNSAEVEKIVTDEKNNREKIALEKNKDKVKEACSKHLKMASYCTTQVERNACLFCKARKLDDKFYQKLRGQFPDAVFWQELGGIFRQLQKQAAEIYNQSLIELYYEIFIKGKGITNASRVEHYLSDVCYTRAAELFKNAAIASGLRGKVKSNFRLKELKNMKSGLPTTKSDNFPIPLVKQKGGQYTGFEIGSHNDDFIIKIPFGRWQAKKEIDKYRPWEKFDFEQVRKSPKPISLLLSTQRRKRNRGWSKDEGTEAEIRKVMNGDYQTSYIEVKRGSKIGEKSAWMLNLSIDVPKIDKGVDPSIIGGIDVGVKSPLVCAINNAFSRYSISDNDLFRFNKKMFARRRILLGKNRHKRAGHGVKNKLKPITILTEKSGRFRKKLIERWACEIADFFIKNKVGTVQMENLESMKRKEDSYFNIRLRGFWPYAEMQNRIEFKLKQYGIKIRKVAPNNTSKTCSKCGHLNNYFNFEYRKKDKFPHFKCEKCNFKEDADYNAALNISNPKLKSTKEEP

SEQ ID NO: 1573 - protein, 726 aa, synthetic construct
SEDEFSHEYWMRHALTLAKRARDGREVPVGAVLVLNNRVIGEGWNRAIGLHDPTAHAEIMALRQGGLVMQNYRLIDATLYVTFEPCVMCAGAMVHSRIGRVVFGVRNSKRGAAGSLMNVLDYPGMNHRVEITEGILVDECAALLCDFYRMPRQVLNAQKKAQSSISSGGSSGGSSGSVTPGASGSVTPKSSGGSSAGSTKDTITKTLKLRIVRPYNSAEVEKIVADEKNNREKIALEKNKDMVKEACSEHLKVTAYCTTQVERNACLFCKARKLDDKFYQKLRGQFPDAVFWQEIGEIFRQLQKQAAEIYNQSLIELYYEIFIKGKGFANASSVEHYLSDVCYTRAAELFKNAAIASGLRGKVKSNFRLKELKNMKSGLPTTKSDNFPIPLVKQKGGQYTGFEISSHNDDFIIKIPFGRWQVKKEIDKYRPWEKFDFEQVRKSPKPISLLLSTQRRKRNKGWSKDEGTEAEIRKVMNGDYQTSYIEVKRGSKIGEKSAWVLNLSIDVPKIDKGVDPSIIGGIDVGVKSPLVCAINNAFSRYSISDNDLFRFNKKMFARRRILLKKNRHKRAGHGAKNKLKPITILTEKSGRFRKKLIERWACEIADFFIKNKVGTVQMENLESMKRKEDSYFNIRLRGFWPYAEMQNKIEFKLKQYGIEIRKVAPNNTSKTCSKCGHLNDYFNFEYRKKNKFPHFKCEKCNFKEDADYNAALNISNPKLKSTKGEP

SEQ ID NO: 1574 - protein, 726 aa, synthetic construct
SEVEFSHEYWMRHALTLARRARDEGEVPVGAVLVLNNRVIGEGWNRAIGLHDPTAHAEIMALRQGGLVMQNYRLVDATLYVTFEPCVLCAGAMVHSRIGRVVFGVRNSKRGAAGSLMNVLNYPGMNHRVEITEGILADECAALLCDFYRMPRQVFNARKKARSNINSSGSSGGSSGRETPGASGSVTPKSSGGGPSGSAKNTITKTLQLRIVRPYNSAEVEKVVADEKNNREKIALEKNKDKVKEACSKHLKVASYCTTQVERNACPFCKARKLDDKFYQKLRGQFPDAVFWQELGEILRQLQKQAAEIYNQSLIELYYEIFIKGKGITNASRVEHYLSDVCYTRAAELFKNAAIASGLRGKVKSNFRLKELKNMKSGLPTTKSDNFPIPLVKQKGGQYTGFEISSHNDDFIIKIPFGRWQVKKEIDKYRPWEKFDFEQVRKSPKPISLLLSTQRRKRNKGWSKDEGTEAEIRKVMSGDYQTSYIEVKRGSKTGEKSAWMLNLSIDVPKIDKDVDPSIIGGIDVGVKFPLVCAINNALSRYSISDNDLFHFNKKMFARRRILLKKNRHKRAGHGAKNKLKPISILTEKSERFRKKLIERWACEIADFFIRNKVGTVQMENLESMKRREDSYFNIRLRGFWPYAKMLNKIEFKLKQYGIKIRKVAPNNTSKTCSKCGHLNNYFNFEYRKKNKFPHFKCEKCNFKENADYNAALNISNPKLKSTKGEP

SEQ ID NO: 1575 - protein, 725 aa, synthetic construct
SEVEFSHEYWMRHALTLAKRARDGREVPVGAVLVLNNRVIGEGWNRAIGLHDPTAHAEIMALRQGGLVMQNYRLIDATLYVTFEPCVMCAGAMVHSRIGRVVFGVRNSKRGAAGSLMNVLNYPGMDHRVEITEGILADECAALLCDFYRMPHQVFNAQKKAQASINSGGSSGGSSGSVTPGPSESATPESSGGSSGSSAKNTITKTLQLRIVRPYNSAEVEKIVADEKNNREKIALEKNKDKVKEACSKHLKVASYCTTQVERNACLFCKARKLDDKFYQKLRGQFPDAVFWQELGEIFRQLQKQAAEIYNQSLIELYYEIFIKGKGFANASSVEHYLSDVCYTRAAELFKNAAIASGLRGKVKSNFRLKELKNMKSGLPTTKSDNFPIPLVKQKGGQYTGFEISSHNDDFIIKIPFGRWQVKKEIDKYRPWEKFDFEQVRKSPRPISLLLSTQRRKRNKGWSKDEGTEAEIRKVMNGDYQTSYIEVKRGSKIGEKSTWMLSLSIDVPKVDKGVDPRIIGGIDVGVKSPLVCAINNVLSRYSISDNDLFHFNKKMFARRRILLKKNGHKRAGHGAKNKLKPITIMTEKSKRFRRKLIERWACEIADFFIKNKVGTVQMENLESMKRKEDSYFNIRLRGFWPYAEMQNKIEFKLKQYGIVVRKVAPNNTSKTCSQCGHLNNYFNFEYRKKNKFPYFKCEKCNFKENADYNAALNISNPQLKSTGEP

SEQ ID NO: 1576 - protein, 726 aa, synthetic construct
SEVEFSHEYWMRHALTLAKRARDEREVPVGAILVLNNRVIGEGWNRAIGLHDPTAHAEIMALRQGGLVMQNYRLIDATLYVTFEPCVMCAGAMIHSRIGRVVFGVRNNKHGAAGSLVNVLDYPGMNHRVEITEGILADECAALLCDFYRMPRQVFNARKKAQSSISPDGSSGGSSGSETPGTSESATPESSGGSSGGSAKNTITKTLKLRIVRPYNSAEVEKIVADEKNNREKIALEKNKGKVKEACSKHLEVAAYCTTQVERNACLFCKARKLDDKFYQKLRGQFPDAVFWQELGEIFRQLQRQAAEIYNQSLIELYYEIFIKGKGFANASSVEHYLSDVCYTRAAELFKNAAIASGLRGKVRSNFRLKELKNMKSGLPTTKSDNFPIPLVKQKGGQYTGFEISSHNSDFIIKIPFGRWQVKKEIDKYRPWEKFDFEQVRKSPKPISLLLSTQRRKRNKGWSKDEGTEAEIRKVMNGDYRISYIEVKRGSKVGEKSAWMLSLSIDVPKIDKGVDPSIIGGIDVGVKSPLVCAINNAFSRHSISDNDLFHFNKKMFARRRILLKKNRHKRAGHGAKNKLKPISILTGKSKRFRKKLIERWACEIADFFIKNKVGTVQMENLESMKRKEDSYFNIRLRGFWPYAEMQNKIEFKLKQYGIEIRKVAPNNTSKTCSKCGHLNNYFNFEYRKRNKFPHFKCEKCNFKENADYNAALNISNPKLKSTKEEP

SEQ ID NO: 1577 - protein, 726 aa, synthetic construct
SEVEFSHEYWMRHALTLAKRARDEREVPVGAILVLNNRVIGEGWNRAIGLHDPTAHAEIMALRQGGLVMQNYRLIDATLYVTFEPCVMCAGAMIHSRIGRVVFGVRNSKHGAAGSLVNVLNYPGMNHRVEITEGILADECAALLCDFYRMPRRVFNAQKKAQSSINSGGSSGGGSGSETPSTSESATPESSGGGSSGSAKNTITKTLQLRIVRPYNSAEVEKIVADEKNNREKIALEKNKDKVKEACSKHLKVASYCTTQVERNACPFCKARKLDDKFYQKLRGRFPDAVFWQELGEILRQLQKQAAEIYNQSLIELYYEIFIKGKGFANASSVEHYLSDVCYTRAAELFKNAAIASGLRGKVKSNLRLKELKNMRSGLPTTKSDNFPIPLVKQKGGQYTGFEISSHNDDFIIKIPFGRWQVKEEIDKYRPWEKFDFEQVRKNPKPISLLLSTQRRKRNKGWSKDEGTEAEIKKVMNGDYQTSYIEVKRGSKIGEKSAWMLNLSIDVPKIDKGVDPSIIGGIDVGVKSPLVCAINNAFSRYSISDNDLFHFNKKMFARRRILLKKNRHKRAGHGAKNKLKPLTILTGKSKRFRKKLIERWACEIADFFIKNKVGTVQMENLESMKRKEDSYFNTRLRGFWPYAEMQNKIEFKLKQYGIEIRKVAPNNTSKTCSKCGHLNNYFNFEYRKRNKFPRFKCEKCNFKENADYNAALNISNPKLKSPKEEP

SEQ ID NO: 1578 - protein, 726 aa, synthetic construct; identical to SEQ ID NO: 684

SEQ ID NO: 1579 - protein, 726 aa, synthetic construct
SEVEFSHEYWMRHALTLAKRARDEREVPVGAVLVLNNRVIGGGWNRAIGLHDPTAHAEIMALRQGGLVMQNCRLVDATLYVTFEPCVMCAGAMIHSRIGRVVFGVRNNKHGAAGSLVNVLNYPGMNHRVEITEGILADECAALLCDFYRMPRQVFNARKKAQSSINPGGSSGGSSGSETPGTSDSATPESSGGSPGGSAQNTITKTLKLRIVRPYNSAEVEKIVADEKNNREKIALEKNKDKVREACSKHLKVAAYCTTQVERNACLFCKARKLDDKFYQKLRGQFPDAVFWQEIGEIFRQLQKQAAEIYNQSLIELYYEIFIKGKGFANASSVEHYLSDVCYTRAAELFKNAAIASGLRGKVKSNFRLKELKNMKSGLPTTKSDNFPIPLVKQKGGQYTGFEISSHNSDFIIKIPFGRWQVKEEIDKYRPWEKFDFEQVRKNPKPISLLLSTQRRKRNKGWSKDEGTEAEIRKVMNGDYQTSYIEVKRGSKIGEKSAWMLNLSIDVPKIDKGVDPSIIGGIDVGVKSPLVCAINNAFSRYSISDNDLFRFNKKVFARRRILLKKNRHKRAGHGTKNKLKPITMLTEKSGRFRKKLIERWACEIANFFIKNKVGTVQMENLESMKRKEDSYFNIRLRGFWPYAEMQNKIEFKLKQYGIKIRKVAPNNTSKTCSKCGHLNNYFSFEYRKRNKFPHFKCEKCNFKEDADYNAALNISNPKLKSTKEEP

SEQ ID NO: 1580 - protein, 726 aa, synthetic construct
SEVEFSHEYWMRHALTLARRARDEREVPVGAVLVLNNRVIGEGWNRAIGLHDPTAHAEIMALRQGGLVMQNYRLIDATLYVTFEPCVMCAGAMIHSRIGRVVFGVRNSKHGAAGSLVNVLNYPGMNHRVEITEGILADECAALLCDFYRMPRQVFNARKKAQSSINSGGSSGGSSGSETPGTSESAAPESSGGSSGGSAKNTITKTLKLRIVRPYNSAEVEKIVADEKNNRERIALEKNKDKVKEACSKHLKVAAYCTTQVERNACLFCRARKLDDKFYQKLRGQFPDAVFWQEIGEIFRQLQKQAAEIYNQSLIELYYEIFIKGKGFANASSVEHYLSDVCYTRAAELFKNAAIASGLRGKVRSNFRLKELKNMKSGLPTTKSDNFPIPLVKQKGGQYTGFEISSHNDDFIIKIPFGRWQVKEEIDKYRPWEKFDFEQVRKSPKPISLLLSTQRRKRNKGWSKDEGTEAEIRKVMNGDYQTSYIEVKRGSKTGEKSAWMLNLSIDVPKIDKGVDPCIIGGIDVGVKSPLVCAINDAFSRYSISDNDLFHFNKKMFARRRILLKKNGHKRAGHGAKNKLKPITIMTEKSKRFRKKLIERWACEIADFFIKNKVGTVQMENLESMKRKEDSYFNIRLRGFWPYAEMQNKIEFKLKQYGIVVRKVAPNNTSKTCSKCGHLNNYFNFEYRKKNKFPHFKCEKCNFKENADYNAALNISNPKLKSTKEEP

SEQ ID NO: 1581 - protein, 726 aa, synthetic construct
SEDEFSHEYWMRHALTLAKRARDGREVPVGAVLVLNNRVIGEGWNRAIGLHDPTAHAEIMALRQGGLVMQNYRLIDATLYVTFEPCVMCAGALVHSRIGRVVFGVRNSKRGAAGSLMNVLDYPGMGHRVEITEGILADECAALLCDFYCMPRQVFNAQKRAQSSINSGGSSGGSGGSETPGTSESATPESSGGGSSGSAKNTITKTLQLRIVRPYNSAEVEKIVADEKNNREKIALEKNKDKVKEACSEHLKVAAYCTTQVERNACLFCKARKLDDKFYQKLRSQFPDAVFWQELGEIFRQLQKQAAEIYNQGLIELYYEIFIKGKGAANASSVEHYLSDVCYTRAAELFKNAAIASGLRNKIKSNFRLKELKNMKSGLPTTKSNNFPIPLVKQKGGQYAGFEISNHNGDFIIKIPFGRWQAKKEINKHRPWEKFDFEQVRKSPKPISLLLSTQRRKRNKGWSKDEGTEAEIRKVMNGDYQTSYIEVKRGSKIGEKSAWMLNLSIDVPKIDKGVDPSIIGGIDVGVKSPLVCAINNALSRYSISDNDLFHFNKKMFARRRILLRKNSHKRAGHGTKNKLKPITIMTEKSKRFRKKLIERWACEIADFFIKNKVGTVQMENLESMKRKEDSYFNIRLRGFWPYAEMQNKIEFKLKQYGIVVRKVAPNNTSKTCSKCGHLNNYFNFEYRKKNKFPHFKCEKCNFKEDADYNAALNISNPKLKSTKGEP

SEQ ID NO: 1582 - protein, 726 aa, synthetic construct
SEVEFSHEYWMRHALTLAKRARDEREVPVGAVLVLNNRVIGEGWNRAVGLHDPTAHAEIMALRQGGLVMQNYRLTDATLYVTFEPCVMCAGAMIHSRIGRVVFGVRNSKRGAAGSLMNVLNYPGMNHCVEITEGILVDECAALLCDFYRMPRQVLSAQKKAQSSVSSGDSSGGSSGSETPGASGSVTPKSSVGSSAGSTKNTITKTLKLRIVRPYNSAEVEKIVADEKNNREKIALEKNKDKVKEACSKHLKVASYCTTQVERNACPFCKARKLDDKFYQKLRGQFPDAVFWQELGEILRQLQKQAAEIYNQSLIELYYEIFIKGRGFANASSVEHYLSDVCYTRAAELFKNAAIASGLRGKVKGNFRLKELKNMKSGLPTTKSDNFPIPLVKQKGGQYTGFEISSHNDDFIIKIPFGRWQVKKEIDKYRPWEKFDFEQVRKSPKPISLLLSTQRRKRNKGWSKDEGTEAEIRKVMNGDYQTSYIEVKRGSKTGEKSAWMLNLSIDVPKIDKGVDPSIIGGIDVGVKSPLVCAINNAFSRYSISDNDLFRFNKKMFARRRILLKKNRHKRAGHGAKNKLKPISILTGKSERFRKKLIERWACEIADFFIKNKVGTVQMENLESMKRKEDSYFNIRLRGFWPYAEMQSKIEFKLKQYGIEIRKVAPNNTSKTCSKCGHLNNYFNFEYRKKNKFPHFKCEKCNFKENADYNAALNISNPKLKSTKEEP

SEQ ID NO: 1583 - protein, 726 aa, synthetic construct
SEVEFSHEYWMRHALTLAKRARDEREVPVGAVLVLNNRVIGEGWNRAIGLHDPTAHAEIMALRQGGLVMQNYRLINATLYVTFEPCVMCAGAMIHSRIGRVVFGVRNSKHGAAGSLMNVLNYPGMNHRVEITEGILADECAALLCDFYRMPCQVFNARKKAQSSVSSGGSSGGSSGSETPGASGSVTPKSSVGSSAGSTKNTITKTLKLRIVRPYNSAEVEKIVADEKNNREKIALEKNKGKVKEACSKHLEVAAYCTTQVERNACLFCKARKLDDKFYQKLRGQFPDAVFWQETGEIFRQLQRQAAEIYNQSLIELYYEIFIKGKGFANASSVEHYLSDVCYTRAAELFKNAAIASGLRGKVKSNFRLKELKNMKSGLPTTKSDNFPIPLVKQKGGQYTGFEISSHNDDFIIKIPFGRWQVKKEINKFRPWEKFDFEQVRKSPKPLSLLLSTQRRKRNKGWSRDEGTEAEIRKVMNGDYQTSYIEVKRGSKIGEKSAWMLNLSIDVPKIDKGVDPSIIGGIDVGVKSPLVCAINNAFSRYSISDNDLFHFNKKMFARRRILLKKTRHKRAGHGAKNKLKPISILTEKSERFRKKLIERWACEIADFFIKNKVGTVQMENLESMKRREDSYFNIRLRGFWPYAKMQNKIEFKLKQYGIEIRKVAPNNTSKTCSKCGHLNNYFSFEYRKKNKFPHFKCEKCNFKEDADYNAALNISNPKLKSTKEEL

SEQ ID NO: 1584 - protein, 726 aa, synthetic construct
SGVEFSHEYWMRHALTLAKRARDEREVPVGAVLVLNNRVIGEGWNRAIGLHDPAAHAEIMALRQGGLVMQNYRLIGATLYVTFEPCVMCAGAMIHSRVGRVVFGVRNNKHGAAGSLVNVLNYPGMNHRVEITEGILADECAALLCDFYRMPRQVFNARKKAQSGINPGGSSGGSSGSETPGTSESATPESSGGSSGGSAKNTITKTLKLRIVRPYNSAEVEKIVADEKNNREKIALEKNKDKVKEACSKHLKVAAYCTTQVERDACLFCKARRLDDKFYQKLRGQFPDAVFWQEVGEIFRQLQKQAAEIYNQSLIELYYEIFIKGKGFANASSVEHYLSDVCYTRAAELFKNAAIASGLRGKVKSNFRLKELKNMKSGLPTTKSDNFPIPLVKQKGGQYTGFEISSHNDDFIIKIPFGRWQVKKEIDKYRPWEKFDFEQVRKSPKPISLLLSTRRRKRNKGWSKDEGTEAEIRKVMNGDYQTSYIEVKRGGKIGEKSAWMLNLSIDVPKIDKGVDPSIIGGIDVGVKSPLVCAINNAFSRYSISDNDLFRFNKKMFARRRILLRKNRHKRAGHGAKNKLKPITIMTEKSKRFRKKLIERWACEIADFFIKNKVGTVQMENLESMKRKEDSYFNIRLRGFWPYAEMQNKIEFKLKQYGIVVRKVAPNNTSKTCSKCGHLNNYFNFEYRKKNKFPHFKCEKCNFKEVADYNAALNISNPKLKSTKEVP

SEQ ID NO: 1585 - protein, 726 aa, synthetic construct
SEVEFSHEYWMRHALTLAKRARDEREVPVGAVLVLNNRVIGEGRNRTIGLHDPTAHAEIMALRQGGLVMQNYRLTDATLYVTFEPCVMCAGAMIHSRIGRVVFGVRNSKRGAAGSLMNVLNYPGMNHCVEITEGILVDECAALLCDFYRMPRQVLNAQKKAQSSISSGGSSGGSSGSETPGASESATPKSSGGSSASSTKNTITKTLRLRIVRPYNSAEVEKIVADEKNNRERIALEENKDKVKEACSKHLKVASYCTTQVERNACPFCKARKLDDKFYQKLRGQFPDAVFWQELGEILRQLQKQAAEIYNQSLIELYYEIFIKGRGFANASSVEHYLSGVCYTRAAELFKNAAIASGLRGKVKSNFRLKELKNMKSGLPTTKSDNFPIPLVKQKGGQYTGFEISSHNDDFIIKIPFGRWQVKKEIDKYRPWEKFDFEQVRKSPKPISLLLSTRRRKRNKGWSKDEGTEAEIRKVMNGDYQTSYIEVKRGSKTGEKSAWMLNLSIDVPKIDKGVDPSIIGGIDVGVKSPLVCAINNAFSRYSISDNDLFRFNKKMFARRRILLKKNRHKRAGHGAKNKLKPISILTGKSERFRKKLIERWACEIADFFIKNKVGTVQMENLESMKRKEDSYFNIRLRGFWPYAEMQNKIEFKLKQYGIEIRKVAPNNTSKTCSKCGHLNNYFNFEYRKKNKFPHFKCEKCSFKENADYNAALNISNPKLKSTKEEP

SEQ ID NO: 1586 - protein, 726 aa, synthetic construct
SEDEFSHEYWMRHALTLAKRARDGREVPVGAVLVLNNRVIGEGWNRAIGLHDPTAHAEIMALRQGGLVMQNYRLIDATLYVTFEPCVMCAGAMVHSRIGRVVFGVRNSKRGAAGSLMNVLDYPGMGHRVEITEGILADECAGLLCDFYCMPRQVFNAQKRAQSSISSGGSSGGSGGGETPGASESVTPKNSGGSSASSTKNTITKTLKLRIVRPYNSAEVEKIVADEKNSREKIALEKNKDKVKEACREHLRVAAYCTTQVERSACLFCKARKLDDKFYQKLRGQFPDAVFWQELGEIFRQLQKQAAEIYNQSLIELYYEIFIKGKGFANASSVEHYLSDVCYTRAAELFKNAAIASGLRGKVKSNFRLKELKNMKSGLPTTKSDNFPIPLVKQKGGQYTGFEISNHNGDFIIKIPFGRWQVKKEINKHRPWEKFDFEQVRKSPKPISLLLSTQRRKGNKGWSKDEGTEAEIRRVMNGDYQTSYIEVKRGSKIGEKSAWMLNLSIDVPKIDKGVDPSIIGGIDVGVKSPLVCAINNALSRYSISDNDLFHFNKKMFARRRILLRKNRHKRAGHGARNKLKPITVLTEKCERFRKKLIERWACEIANFFIKNKVGTVQMENLESMKRREDSYFNIRLRGFWPYAEMQNKIEFKLKQYGIEIRKVAPNNTSKTCSKCGHLNNYFNFEFRKKNKFPHFKCEKCNFKENADYNAALNISNPKLKSTKEEP

SEQ ID NO: 1587 - protein, 726 aa, synthetic construct
SEDEFSHEYWMRHALTLAKRARDGREVPVGAVLVLNNRVIGEGWNRTTGLHDPTAHAEIIALRQGGLVMQNHRLVDATLYVTFEPCVMCAGAMIHSRIGRVVFGVRNSKRGAAGSLMNVLNYPGMDHCVEITEGILVDECAALLCDFYRMPRQVLNAQKKAQSSISSGGSSGGSSGSETPGTSESPTPESSGGSSGGSAKNTITKTLQLRIVRPYNSAEVEKIVTDEKNNREKIALEKNKDKVKEACGKHLKMASYCTTQVERNACLFCKARKLDDKFYQKLRGQFPDAVFWQELGGIFRQLQKQAAEIYNQSLIELYYEIFIKGKGITNASRVEHYLSDVCYTRAAELFKNAAIASGLRSKVRSNFRLKELRNMKSGLPTTKSDNFPIPLVKQKGGQYTGFEISSHNSDFIIKIPFGRWQVKEEIDKYRPWEKFDFEQVRKSPKPISLLLSTQRRKKNKGWSKDEGTEAEIRRVMNGDYQTSYIEVKRGSKIGEKSAWMLNLSIDVPKIDKGVDPSIVGGIDVGVKSPLVCAINNAFSRYSISDNELFHFNKKMFARRRILLKKNWHKRAGHGAKNKLKPISILTEKSERFRKKLIERWACEIANFFIKNKVGTVQMENLEGMKRKEDSYFNIRLRGFWPYAEMQNKIEFKLKQYGIEIRKVAPNNTSKTCSKCGHLNNYFNFEYRKKNKFPHFKCEKCNFREDADYNAALNISNPKLKSTKEEP

SEQ ID NO: 1588 - protein, 726 aa, synthetic construct
SEVEFSHEYWMRHALTLAKRARDEREVPVGAVLVLNNRVIGEGWNRAIGLHDPTAHAEIMALRQGGLVMQNYRLVDATLYVTFEPCVLCAGAMVHSRIGRVVFGVRNSKRGAAGSLMNVLNYPGMNHRVEITEGILADECAALLCDFYRMPRQVFNARKKARSNINSGGSSGGSSGSETPGTSESPTPESSGGSPGGSAKNTITKTLKLRIVRPYNSTEVEKIVADEKNNREKIALEKNKDKVKEACSKHLKVAAYCTTQVERNACLFCKARKLDDKFYQKLRGQFPDAVFWQEIGEIFRQLQKQAAEIYNQSLIELYYEIFIKGRGFANASSVEHFLSDVCYTRAAELFKNAAIASGLRGKVKSNFRLKELKNMKSGLPTTKSDNFPIPLVKQKGGQYTGFEISSHNDDFIIKIPFGRWQVKKEVNKYRPWEKFDFEQVRKSPKPISLLLSTQRRKRNKGWSKDEGTEAEIRKVMNGDYQTSCIEVKRGSKIGEKSAWMLNLSIDVPKIDKGVDPSIVGGIDVGVKSPLVCAINNAFSRHSISDNDLFHFNKKMFARRRILLKKNRHKRAGHGVKNKLKPISILTEKSKRFRKKLIERWACEIADFFIKNKVGTVQMENLESMKRKEDSYFNIRLRGFWPYAEMQNKIEFKLKQYGIKIRKVAPNNTSKTCSKCGHLNNYFDFEYRKRNKFPHFKCEECNFKENADYNAALNISNPKLKNTKGEP

SEQ ID NO: 1589 - protein, 726 aa, synthetic construct
SEVEFSHEYWMRHALTLAKRARDEREVPVGAVLVLNNRVIGEGWNRAIGMHDPTAHAEIMALRQGGLVMQNYRLVDATLYVTFEPCVLCAGAMVHSRIGRVVFGVRNSKRGAAGSLMNVLNYPGMNHRVEVTEGILADECAALLCDFYRMPRQVFNARKKARSNINSGGSSGGSSGSETLGTREGATPESSGGSSGGSAKNTITKTLKLRIVRPYNSAEVEKIVVDEKNNREKVALEKNKDKVKEACSEHLKVAAYCTTQVERSACLFCKARKLDDGFYQKLRGQFPDAVFWQEIGEIFRQLQKQAAAIYNQSLIELYYEILIKGKGFANASSVEHYLSDVCYTRAAELFKNAAIASGLRGKVKSNFRLKELKNMKSGLPTTKSDNFPIPLVKQKGGQYTGFEISNHNGDFIIKIPFGRWQVKKEIDKYRPWEKFDFEQVRKSPKPISLLLSTQRRKRNKGWSKDEGTEAEIKKVMNGDYQTSYIEVKRGSKIGEKSAWMLNLSIDVPKIDKGVDPSIIGGIDVGVKSPLVCAINNAFGRHSISDNDLFHFNKKMFARRRILLKKNRHKRAGHGAKNKLKPISILTEKSKRFRKKLIERWACEIADFFIKNKVGTVQMENLESMKRKEDSYFNIRLRGFWPYAEMQNKIEFKLKQYGIEIRKVAPNNTSKTCSKCGHLNNYFNFEYRKKNKFPHFKCEKCSFKENADYNAALNISNPKLKSTKEEP

SEQ ID NO: 1590 - protein, 726 aa, synthetic construct
SEVEFSHEYWMRHALTLAKRARDEREVPVGAVLVLNNRVIGEGWNRTTGLHDPTAHAEIMALRQGGLVMQNHRLVDATLYVTFEPCVMCAGAMIHSRIGRVVFGVRNSKRGAAGSLTNVLNYPGMNHRVEITEGILVGECAALLCDFYRMPRQVFNAQKKAQSTINSGGSSGGSSGSETQGTSEGPTPESSGGSPGGSAKNTITKTLKLRIVRPYNSAEVEKIVADEKNNREKIALEKNKDKVKEACSKHLKVAAYCTTQVERNACLFCKARKLDDKFYQKLRGQFPDAVFWQEIGEVFRQLQKQAAEIYNQSLIELYYEIFIKGKGFANASSVEHYLSDVCYTRAAELFKNAAIASGLRGKVKSNFRLKELKNMKSGLPTTKSDNFPIPLVKQKGGQYTGFEISSHNDDFIIKIPFGRWQAKKEINKFRPWEKFDFEQVRKSPKPISLLLSTQRRKRNKGWSRDEGTEAEIRKVMNGDYQTSYIEVKRGSKIGEKSAWMLNLSIDVPKIDKGVDPSIIGGIDVGVKSPLVCAINNAFSRYSISDNDLFHFNKKMFARRRILLKKNGHKRAGHGAKNKLKPITIMTEKSKRFRKKLIERWACEIADFFIKNKVGTVQMENLESMKRKEDSYFNIRLRGFWPYAEMQNKIEFKLKQYGIEIRKVAPNNTSKTCSKCGHLNNYFNFEYRKMNKFPHFKCEKCNFKENADYNAALNISNPKLKSTKEEP

SEQ ID NO: 1591 - protein, 726 aa, synthetic construct
SEVEFSHEYWMRHALTLAKRARDEREVPVGAILVLNNRVIGEGWNRAIGLHDPTAHAEIMALRQGGLVMQNYRLIDATLYVTFEPCVMCAGAMIHSRIGRVVFGVRNNKHGAAGSLVNVLNYPGMNHRVEITEGILANECAALLCDFYRMPRQVFNARKKAQSSINPSGSSGGSSGSVTPGTSESATPESSGGGSGGSAKNTITKTLQLRIVRPYNSAEVEKIVTDEKNNREKIALEKNKDKVKEACSKHLKMASYCTTQVERNACLFCKARKLDDKFYQKLRGQFPDAVFWQELGGIFRQLQKQAAEIYNQSLIELYYEIFIKGKGITNASRVEHYLSDVCYTRAAELFKNAAIASGLRSKVRSNFRLKELKNMKSGLPTTKSDNFPIPLVKQKGGQYTGFEISSHNSDFIIKIPFGRWQEKEEIDKYRPWEKFDFEQVRRSPKPISLLLSTQRRKKNKGWSKDEGTEAEIRRVMNGDYQTSYIEVKRGSKIGEKSAWMLNLSIDVPKIDKGVDPSIIGGIDVGVKSPLVCAINNAFSRYSISDNDLFHFNKKMFARRRILLKKNRHKRAGHGAKNKLKPISILTEKSERFRKKLIEKWACEIADFFVKNKVGTVQMENLESMKRKEDSYFNIRLRGFWPYAEMQNRIEFKLKQYGIEIRKVAPNNTSKTCSKCGHLNNYFNFEYRKKNKFPHFKCEKCNFKENADYNAALNISNPKLKSTKEGP

SEQ ID NO: 1592 - protein, 726 aa, synthetic construct
SEDEFSHEYWMRHALTLAKRARDGREVPVGAVLVLNNRVIGEGWNRAIGLHDPTAHAEIMALRQGGLVMQNYRLIDATLYVTFEPCVMCAGAMVHSRIGRVVFGVRNSKRGAAGSLMNVLDHPGMGHRVEITEGILADECAALLCDFYCMPRQVFNAQKRAQPSIDSGGSSGGSSGSETPGTSESATPESSGGGSSGSAKNTITKTLQLRIVRPYNSAEVEKIVADEKNNREKIALEKNKDKVKEACSKHLKVASYCTTQVERNACPFCRARKLDDKFYQKLRGQFPDAVFWQELGEILRQLQKQAAEIYNQSLIELYYEIFIKGRGFANASSVEHYLSDVCYTRAAELFKNAAIASGLRSKVRSNFRLKELKNMKSGLPTTKSDNFPIPLVKQKGGQYTGFEISSHNSDFIIKIPFGRWQVKEEIDKYRPWEKFDFEQVRKSPKPISLLLSTQRRQKNKGWSKDEGTEAEIRRVMNGDYQTSYIEVKRGSKIGEKSTWMLNLSIDVPKIDKGVDPSIVGGIDVGVKSPLVCAINNSFSRYSICDNDLFRFNKKMFARRRILLKKNRHKRAGHGAKNKLKPISILTEKSKRFRKKLIERWACEIADFFIKNKVGTVQMENLESLKRKEDSYFNIRLRGFWPYAEMQNRIEFKLKQYGIEIRKVAPNNTSKTCSKCGHLNNYFNFEYRKKNKFPHFKCEKCNFKEDADYNAALNISNPRLKGTKEEP

SEQ ID NO: 1593 - protein, 726 aa, synthetic construct
SEAELSHEYWMRRALTLAERARDEREVPVGAVLVLNNRVIGVGWNRAIGLHDPTAHAEIMALRQGGLVTQNYRLIDATLYVTFEPCIMCAGAMIHSRIGRVVFGVRNSKRGAAGSLMNVLDYPGMNHRVEITEGILAGECAALLCDFYRMPRQVFNAQKRAQSNINPGGSSGDSSGSETPGTSESPTPESSGGSSGGSAKSTITKTLKLRIVRPYNSAEVEKIVADEKNNREKIALEKNKGKVKEACSKHLKVAAYCTTQVERNACLFCKARKLDDKFYQKLRGQFPDAVFWQELGGIFRQLQKQAAEIYNQSLIELYYEIFIKGKGITNASRVEHYLSDVCYTRAAELFKNAAIASGLRGKVKSNFRLKELKNMRSGLPTTKSDNFPIPLVKQKGGQYAGFEICSHNDDFIIKIPFGRWQVKKEIDKYRPWEKFDFEQVRKSPKPISLLLSTQRRKRNKGWSKDEGTEAEIKKVMNGDYQISYIEVKRGSKVGEKSSWMLNLSVDVPKIDKGVDPSIIGGIDVGVKSPLVCAINNALSRYSISDNDLFHFNKRMFARRRILLRRNRHKRAGHGAKNKLKPITILTEKSVRFRKKLIERWACEIADFFIKNKVGTVQMENLESMKRKEDSYFNIRLRGFWPYAEMQNKIEFKLKQYGIEIRRVAPNNTSRTCSKCGHLNNYFNFEYRRKNKFPHFKCEKCNFKEDADYNAALNISNPKLKSTKEEP

SEQ ID NO: 1594 - protein, 726 aa, synthetic construct
SEVEFSHEYWMRHALTLAKRARDGREVPVGAVLVLNNHVIGEGWNRAIGLHDPTAHAEIMALRQGGLVMQNYRLIDATLYVTFEPCVMCAGAMVHSRIGRVVFGVRNSKRGAAGSLMNVLDYPGMGHRVEITEGILADECAALLCDFYCMPRQVFNAQKRAQSSINSGGSSGGSSGSETPGTSESATPESSGGGSSGSAKNTITKTLQLRIVRPYNSAEVEKIVADEKNNREKIALEKNKDKVREACNKHLKVASYCTTQVERNACPFCKARKLDDKFYQKLRGQFPDAVFWQELGEILRQLQKQAAEIYNQSLIELYYEIFIKGRGFANASSVEHYLSDVCYTRAAELFKNAAIASGLRGKVKSNFRLKELKNMKSGLPTTKSDNFPIPLVKQKGGQYTGFEISSRNDDFIIKIPFGRWQAKKEIDRYRPWEKFDFEQVRKSPKPISLLLSTRRRKRNKGWSKDEGTEAEIRKVMNGDYQTSYIEVKRGSKIGEKSAWMLNLSIDVPKIDKGVDPGIIGGIDVGVKSPLVCAINNASSRYSISDNDLFHFNKKMFARRRILLKKNRHKRAGHGAKNKLKPITIMTEKSKRFRKKLIERWACEIADFFIKNKVGTVQMENLESMKRKEDGYFNIRLRGFWPYAEMQNKIEFKLKQYGIEIRKVAPNNTSKTCSKCGHLNNYFNFEYRKMNKFPHFKCEKCNFKEDADYNAALNISNPKLKSTKEEP

SEQ ID NO: 1595 - protein, 726 aa, synthetic construct
SEVEFSHEYWMRHALTLAKRARDEREVPVGAILVLNNRVIGEGWNRAIGLHDPTAHAEIMALRQGGLAMQNYRLIDATLYVTFEPCVMCAGAMIHSRIGRVVFGVRNSKHGAAGSLVNVLNYPGMNHRVETTEGILADECAALLCDFYRMPRQVFNARKKAQSSINPGGLSGGSSGSVTPGTSESATPGSSGGSSGVSAKNTITKTLKLRIVRPYNSAEVEKIVADEKNNREKIALEKNKDKVKEACSKHMKVAAYCTTQVERNACLFCKARRLDDKFYQKLRGQFPDAVFWQEIGDIFRQLQKQAAEIYNQSLIELYYEIFIKGKGFANASSVEHYLSDVCYTRAAELFKNAAIASGLRGKVKSNFRLKELKNMKSGLPTTKSDNFPIPLVKQKGGQYTGFEISSHNDDFIIKIPFGRWQVKKEIDKYRPWEKFDFEQVRKSPKPISLLLSTQRRKRNKGWSKDEGTEAEIRKVMNGDYQTSYIEVKRGSRTGEKSAWMLNLSIDVPKIDKGVDPSIIGGIDVGVKSPLVCAINNAFSRYSISDNDLFRFNKKMFARRRILLKKNRHKRAGHGAKNKLKPISILTGKSERFRKKLIERWACEIADFFIKNKVGTVQMENLESMKRKEDSYFNIRLRGFWPYAEMQNKIEFKLKQYGIEVRKVAPNNTSKTCSKCGHLNNYFNFEYRKKNKFPHFKCEKCNFRENADYNAALNISNPKLKSTKEEP

SEQ ID NO: 1596 - protein, 726 aa, synthetic construct
SEVEFSHEYWMRHALTLAKRARGEREVPVGAILVLNNRVIGEGWNRAIGLHDPTAHAEIMALRQGGLVMQNYRLIDATLYVTFEPCVMCAGAMVHSRIGRVVFGVRNSKRGAAGSLMNVLNYPGMNHRVEITEGILADECAALLCDFYRMPRQVFNAQKKARSNINSGGSSGGSSGSETPGTSESATPESSGGGSSGSAKNTITKTLQLRIVRPYNSAEVEKIVADEKNNREKIALEKNKDKVKEACSKHLKVASYCTTQVERNACPFCKARKLDDKFYQKLRGQFPDAVFWQEIGEIFRQLQKQAAETYNQSLIELYYEIFIKGKGFANASSVEHYLSDVCYTRAAELFKNAAIASGLRGKVKSNFRLKELKNMKSGLPTTKSDNFPIPLVKQKGGQYTGFEISSHNDDFIIKIPFGRWQVKEEIDKYRPWEKFDFEQVRKSPKPISLLLSTQRRKRNKGWSKDEGTEAEIRKVMNGDYQTSYIEVKRGSKTGEKSTWMLNLSIDVPKIDKGVDPSIIGGIDVGVKSPLVCAINNAFSRYSISDNDLFRFNKKVFARRRILLKKNRHKRAGHGTKNKLKPITILTEKSGRFRKKLIERWACEIANFFIKNKVGTVQMENLESMKRKEDSYFNIRLRGFWPYAEMQNKIEFKLKQYGIKIRKVAPNNTSKTCSKCGHLNNYFSFEYRRKNKFPHFKCEKCNFKEDADYNAALNISNPKLKSTKEEP

SEQ ID NO: 1597 - protein, 726 aa, synthetic construct
SEVEFSHEYWMRRALTLAKRARDEREVPVGAVLVLNNRVIGEGWNRAIGLHDPTAHAEIMALRQGGLVMQNYRLTDATLYVTFEPCVMCAGAMIHSRIGRVVFGIRNSKRGAAGSLMNVLNYPGMNHCVKITEGILVDECAALLCDFYRMPRRVLNAQKRAQSSISSGGSSGGSSGSGTPGASESVTPKSSVGSSAGSTKNTITKTLKLRIVRPYNSAEVEKIVADEKNNREKIALEKNKDKVKEACSKHLKVAAYCTTQVERSACLFCKARKLDDKFYQKLRGQFPDAVFWQEIGEIFRQLQKQAAEIYNQSLIELYYEIFIKGKGFANASSVEHYLSDVCYTRAAGLFKNAAIASGLRGKVKSNFRLKELKNMKSGLPTTKSDNFPIPLVKQKGGQYTGFEISSHNDDFIIKIPFGRWQVKKEINKFRPWEKFDFEQVRKNPKPISLLLSTQRRKGNKGWSKDEGTEAEIRKVMNGDYQTSYIEVKRGSKIGEKSAWMLSLSIDVPKIDKGVDPSIIGGIDVGVKSPLVCAINNAFNRYSISDNNLFHFNKKMFARRRILLKKNRHKRAGHGAKNKLKPISILTEKSERFRKKLIERWACEIADFFIRNKVGTVQMEDLEGMKRKEDSYFNIRLRGFWPYAEMQNKIEFKLKQYGIEVRKVAPNNTSKTCSKCGHLNNYFSFEYRKKNKFPHFKCEKCNFKEDADYNAALNISNPKLKGTKEEL

SEQ ID NO: 1598 - protein, 726 aa, synthetic construct
SEVEFSHEYWMRHALTLAKRARDEREVPVGAILVLNNRVIGEGWNRAIGLHDPTAHAEIMALRQGGLVMQNYRLTDATLYATFEPCVMCAGAMIHSRIGRVVFGVRNSKHGAAGSLMNVLNYPGMNHRVEITEGILADECAGLLCDFYRMPRQVFSARKKAQSSINPGGSSGGSSGSETPGTSESATPESSGGSSGSSAKNTITKTLKLRIVRPYNSAEVEKIVADEKNNREKIALEKNEDKVKEACSKHLKVAAYCTTQVGRNACLFCKARRLDDKFYQKLRGQFPDAVFWQEIGEIFRQLQKQAAEVYNQSLVELYYEILIKGKGIANASSVEHYLSDVCYTRAAELFKNAAIASGLRNKIKSNFRLKELRNMKSGLPTTKSDNFPIPLVRQKGGQYTGFEISNHDGDFIIKIPFGRWQVKKEINKHRPWEKFDFEQVRKSPKPISLLLSTQRRKKNKGWSKDEGTEAEIRRVMNGDYQTSYIEVKRGSKIGEKSAWMLNLSIDVPKIDKGVDPSIIGGIDVGVKSPLVCAINNAFSRYSISDNDLFHFNKKVFARRRILLKKNKHKRAGHGAKNKLKPISILTEKSKRFRKKLIERWACEIADFFIKNKVGTVQMENLESMKRREDSYFNIRLRGFWPYAEMQNKIEFKLKQYGIKIRKVAPNNTSKTCSKCGHLNNYFNFEYRRKNKFPHFKCEKCNFKENADYNAALNISNPKLKSTKEGP

SEQ ID NO: 1599 - protein, 726 aa, synthetic construct
SEVEFSHEYWMRHALTLAKRARDEREVPVGAVLVLNNRVIGEGWNRAIGLHDPTAHAEIMALRQGGLVMQNYRLTDATLYVTFEPCVMCAGAMIHGRIGRVVFGVRNSKHGAAGSLMNVLNYPGMNHRVEITEGILADECAALLCDFYRMPHRVLNARKKAQSSINPGGSSCGSSGSETPGTSESATPESSGGSSGGSAKNTITKTLKLRIVRPYNSAEVEKIVADEKNNRERIALEKNKDKVKEACSKHLKVAAYCTTQVERNACLFCKARRLDDKFYQKLRGQFPDAVFWQEIGEIFRQLQKQAAEIYNQSLIELYYEIFIKGKGFANASSVEHYLSDVCYTRAAELFKNAAIASGLRGKVRSNFRLKELKNMKSGLPTTKSDNFPIPLVKQKGGQYTGFEISSHNSDFIIKIPFGRWQVKKEINKYRPWEKFDFEQVRKSPKPISLLLSTRRRKRNKGWSKDEGTEAEIRRVMNGDYQTSYIEVKRGSKIGEKSAWMLNLSIDVPKIDKGVDPSIIGGIDVGVKSPLVCAINNAFSRYSISDNDLFRFNKKVFARRRILLKKNRHKRAGHGTKNKLKPITILTEKSGRFRKKLIERWACEIANFFIKNKVGTVQMENLESMKRKEDSYFNIRLRGFWPYAEMQNKIEFKLKQYGIKIRKVAPNNTSKTCSKCGHLNNYFSFEYRKKNKFPHFKCEKCNFKEDADYNAALNISNPKLKSTKEGP

SEQ ID NO: 1600 - protein, 726 aa, synthetic construct
SEVEFSHEYWMRHALTLAKRARDEREVPVGAILVLNNRVIGEGWNRAIGLHDPTAHAEIMALRQGGLAMQNYRLADATLYVTFEPCVMCAGAMVHSRIGRVVFGVRNSKRGAAGSLMNVLNYPGMSHCVEITEGILVDECAALLCDFYRMPRQVLNAQKKAQSSISSGGSSGGSGGGETPGASESVTPKSSGGSSAGSTKDTITKTLKLRIVRPYNSAEVEKIVADEKNNREKIALEKNKDKVKEACSKHLKVASYCTTQVERNACPFCKARKLDDKFYQKLRGQFPDAVFWQELGEILRQLQKQAAEIYNQSLIELYYEIFIKGKGFANASSVEHYLSDVCYTRAAELFKNAAIASGLRGKVKSNFRLKELKNMKSGLPTTKSDNFPIPLVRQKGGQYTGFEISSHNDDLIIKVPFGRWRVKREIDKYRPWEKFDFEQVRKSPKPISLLLSTQRRKRNKGWSKDEGTEAEIRKVMNGDYQTSYIEVKRGSKIGEKSAWMLNLSIDVPKIDKGVDPSIIGGIDVGVKSPLVCAINNAFSRYSISDNDLFHYNKKMFARRRILLKKNRHKRAGHGAKNKLRPISILTEKSKRFRKKLIERWACEIADFFIKNKVGTVQMENLESMKRKEDSYFNIRLRGFWPYAEMQNKIEFKLKQYGIEIRKVAPNNTSKTCSKCGHLNSYFNFEYRKKNKFPHFKCEKCNFKENADYNAALNISNPKLKSTKEEP

SEQ ID NO: 1601 - protein, 726 aa, synthetic construct
SEVEFSHEYWMRHALTLAKRARDEREVPVGAVLVLNNRAIGEGWNRAIGLHDPTAHAEIMALRQGGLVMQNYRLVDATLYVTFEPCVLCAGAMIHSRIGRVVFGVRNSKRGAAGSLMNVLNYPGMNHRVEITEGILADECAALLCDFYRMPRQVFNARKKARSNINSGGSSGGSSGSETLGTREGATPESTGGSSGGSAKNTITKTLKLRIVRPYNSAEVEKIVADEKNNRERIALEKNKDKVKEACSKHLKVAAYCTTQVERNACLFCKARKLDDKFYQKLRGQFPDAVFWQEIGEIFRQLQKQAAEIYNQSLIELYYEIFIKGKGFANASSVEHYLSGVCYTRAAELFKNAAIASGLRGKVKSNFRLKELKNMKSGLPTTKSDNFPIPLVKQKGGQYTGFEISSHNDDFIIKIPFGRWQVKEEIDKYRPWEKFDFEQVRKNPKPISLLLSTQRRKGNKGWSKDEGTEAEIRKVMNGDYQTSYIEVKRGSKIGEKSAWMLNLSIDVPKIDKGVDPSIIGGIDVGVKSPLVCAINNAFSRYSISDNDLFHFNKKMFARRRILLKKNRRKRAGHGAKNKLKPISILTEKSKRFRKKLIERWACEIADFFIKNKVGTVQMENLESMKRKEDSYFNIRLRGFWPYAEMQNKIEFKLKQYGIEIRKVAPNNTSKTCSKCGHLNNYFNFEYRKKNKFPHFKCEKCNFKENADYNAALNISNPKLKNTKEEP

SEQ ID NO: 1602 - protein, 726 aa, synthetic construct
SEVEFSHEYWMRHALTLAKRARDEREVPVGAVLVLNNRVIGEGWNRMTGLHDPTAHAEIMALRQGGLVMQNHRLVDATLYVTFEPCVMCAGAMIHSRIGRVVFGVRNSKRGAAGSLTNVLNYPGMNHCVEITEGILVDECAALLCDFYRMPRQVLNAQKKAQSSISSGGSSGGSSGSETSGASGSVTPKSSGGSSGGSAKNTITKTLKLRIVRPYNSAEVEKIVADEKNNREKIALEKNKGKVKEACSKHLEVAAYCTTQVERNACLFCKARKLDDKFYQKLRGQFPDAVFWQELGEIFRQLQKQAAEIYNQSLIGLYYEIFIKGKGFANASSVEHYLSDVCYTRAAELFKNAAIASGLRGKVKSNFRLKELKNMKSGLPTTKSDNFPIPLVKQKGGQYTGFEISSHNDDFIIKIPFGRWQVRKEIDRYRPWEKFNFEQVRKSPKPISLLLSTQRRKKNKGWSKDEGTEAEIRRVMNGDYQTSYIEVKRGSKIGEKSAWMLNLSIDVPKIDKGVDPSIVGGIDVGVKSPLVCAINNAFSRYSISDNDLFHFNKKMFARRRILLKKNRHRRAGHGAKNKLKPITILTEKSVRFRKKLIERWACEIADFFIKNKVGTVQMENLESMKRKEDSYFNIRLRGLWPYAEMQNKIEFKLKQYGIEIRKVAPNNTSKTCSKCGHLNNYFNFEYRRKNKFPYFKCEKCNFKENADYNAALNISNPQLKSTKGEP

SEQ ID NO: 1603 - protein, 726 aa, synthetic construct
SEVEFSHEYWMRHALTLAKRARDEREVPVGAVLVLNNRVIGEGWNRAIGLHDPTAHAEIMALRQGGLVMQNYRLIDATLYVTFEPCVMCAGAMIHSRIGRVVFGVRNSKHGAAGSLVNVLNHPGMNHRVEITEGILADECAALLCDFYRMPRQVFNARKKAQSSINPGGSSGGSSGSVTPGTSESATPESSGGGFGGSAKNTITKTLQLRIVRPYNSAEVEKIVADEKNNREKIALEKNKDKVKEACSKHLKVAAYCTTQVERNACLFCRARKLDDKFYRKLRGQFPDAVFWQEIGEIFRQLQKQAAEIYNQSLIELYYEIFIKGKGFANASSVEHYLSDVCYTRAAELFKNAAIASGLRGKVKSNFRLKELKNMKSGLPTTKSDNFPIPLVKQKGGQYTGFEISSHNDDFIIKIPFGRWQVKKEIDKYRPWEKFDFEQVRKSPKPISLLLSTQRRKRNKGWSKDEGTEAEIRKVMNGDYQTSYIEVKRGSKTGEKSAWMLNLSIDVPKIDKGVDPSIIGGIDVGVKSPLVCAINNAFSKYSISDNDLFRFNKKMFARRRILLKKNRHKRAGHGAKNKLKPISILTGKSERFRKKLIERWACEIADFFIKNKVGTVQMENLESMKRKEDSYFNIRLRGFWPYAEMQNKIEFKLKQYGIEIRKVAPNNTSKTCSKCGHLNNYFNFEYRKKNKFPHFKCEKCNFKENADYNAALNISNPKLKSTKEKP

SEQ ID NO: 1604 - protein, 726 aa, synthetic construct
SGVEFSHEYWMRHALTLAKRARDEREVPVGAVLVLNNRVIGVGWNRAIGLHDPTAHAEIMALRQGGLVTQNYRLIDATLYVTFEPCVMCAGAMIHSRIGRVVFGVRNSKRGAAGSLMNVLNYPGMNHRVEITEGILVDECAALLCDFYCMPRQVFNAQKRAQSSINSGGSSGGSSGSETPGTSESATPESSGGGSSGSAKNTITKTLKLRIVRPYNSAEVEKIVADEKNSREKIALERNKDKVKEACSEHLKVAAYCTTQVERNACLFCKARKLDDRFYQKLRGQFPDAVFWQETGEIFRQLQRQAAEIYNRSLIELYYEIFIKGKGFANASSVEHYLSDVCYTRAAELFKNAAIASGLRGKVKSNFRLKELKNMKSGLPTTKSDNFPIPLVKQKGGQYTGFEISSHNDDFIIKIPFGRWQVKKEIDKYRPWEKFDFEQVRKSPKPISLLLSTQRRKRNKGWSKDEGTEAEIRKVMNGDYQTSYIEVKRGSKTGEKSAWMLNLSIDVPKIDKGVDPSIIGGIDVGVKSPLVCAINNAFSRYSVSDNDLFRFNKKMFARRRILLKKNKHKRAGHGAKNKLKPITILTEKSGRFRKKLIERWACEIADFFIKNKVGTVQMENLESMKRKEDSYFNIRLRGFWPYAEMQNKIEFKLKQYGIKIRKVAPNNTSKTCSKCGHLNNYFSFEYRKKNKFPHFKCEKCNFKEDADYNAALNISNPKLRSTKEEP

SEQ ID NO: 1605 - protein, 726 aa, synthetic construct
SEVEFSHEYWMRHALTLAKRARDEREVPVGAVLVLNNRIIGEGWNRAIGLHDPTAHAEIMALRQGGLVMQNHRLVDATLYVTFEPCVLCAGAMVHSRIGRVVFGVRNGKRGAAGSLMNVLNYPGMNHRVEITEGILADECAALLCDFYRMPRQVFNARKMARSNINSGGSSGGGSGSETPSTSENTTPESSGGSSGGPAKNTITKTLKLRIVRPYNSAEVEKIVADEKNNREKTALERNKDKVKEACSKHLKMAAYCTTQVERNACLFCKARKLDDKFYQKLRGQFPDAVFWQEIGEIFRQLQKQAAEIYNQSLIELYYEIFIKGKGFANASSVEHYLSDVCYTRAAELFKNAAIASGLRGKVKSNFRLKELKNMKSGLPTTKSDNFPIPLVKQKGGKYTGFEISSHNDDFIIKIPFGRWQVKEEIDKYRPWEKFDFEQVRKSPKPISLLLSTQRRKRNKGWSKDEGTEAEIRKVMNGDYQTSYIEVKRGSKIGEKSAWMLNLSIDVPKIDKGVDPSIIGGIDVGVKSPLVCAINNALSRYSISDNDLFHFNKKMFARRRILLRNNRHKRAGHGAKSKLKPITILTEKGERFRKKLIERWACEIANFFIKNKVGTVQMENLESMKRKEDSYFNVRLRGFWPYAEMQNKIEFKLKQYGIEIRKVAPNNTSKTCSRCGHLNNYFNFEYRRKNKFPHFKCEKCNFKENADYNAALNISNPKLKSTKEEP

SEQ ID NO: 1606 - protein, 726 aa, synthetic construct
SEDEFSHEYWMRHALTLAKRARDGREVPVGAVLVLNNRVIGEGWNRAIGLHDPTAHAEIMALRQGGLVMQNYRLIDATLYVTFEPCVMCAGAMVHSRIGRVVFGVRNSKRGAAGSLMNVLDYPGMGHRVEITEGILADECAALLCDFYCMPRQVFNAQKRAQSSINSGGSSGGSSGSETPGASESTTPESSGGSSGGSAKNTITKTLQLRIVRPYNSAEVEKIVTDEKNNREKIALEKNKDKVKEACSKHLKMASYCTTQVEGNACLFCKARKLDDKFYQKLRGQFPDAVFWQELGGIFRQLQKQAAEIYNQSLIELYYEIFIKGKGITNASRVEHYLSDVCYTRAAELFKNAAIASGLRSKVRSNFRLKELKNMKSGLPTTKSDNFPIPLVKQKGGQYTGFEISSHNSDFIIKIPFGRWQVKEEIDKYRPWEKFDFEQVRKSPKPISLLLSTQRRKKNKGWSKDEGTEAEIRRVMNGDYQTSYIEVKRGSKIGEKSAWMLNLSIDVPKIDKGVDPSIIGGIDVGVKSPLVCAINNSSSRYSICDNDLFRFNKKMFARRRILLKKNRHKRAGHGAKNKLKPITILTKKSERFRKKLIERWVCEVADFFIKNKVGTVQMENLESMKRKEDSYFNIRLRGFWPYAEMQNRIELKLKQYGIEIRRVAPNNTSRTCSKCGHLNNYFNFEYRKKNKFPHFKCEKCNFKEDADYNAALNISNPKLRSTKEEP

SEQ ID NO: 1607 - protein, 726 aa, synthetic construct
SEVEFSHEYWMRHALTLAKRARDGREVPVGAVLVLNNRVIGEGWNRAIGLHDPTAHAEIMALRQGGLVMQNYRLIDATLYVTFEPCAMCAGAMVHSRIGRVVFGARNSKRGAAGSLMNVLNYPGMDHRVEITGGILADECAALLCDFYCMPRQVFNAQKRAQSSINPGGSSGGSSGSETPGTSDSATPGSSGGSSGGSAKNTITKTLKLRIVRPYNSAEVEKIVADEKNNREKTALEKNKDKVKEACSEHLKVATYCTTQVERNACLFCKARKLDDKFYQKLRGQFPDAVFWQEIGEIFRQLQKQAAEIYNQSLIELYYEIFIKGKGFANASSVEHYLSDVCYTRAAELFKNAAIASGLRNKTKSNFRLKELRSMKSGLPTTKSDNFPIPLVKQKGGQYTGFEISNHNSDFIIKIPFGRWQAKKEIDKYRPWEKFDFEQVRKSPKPISLLLSTQRRKRNKGWSKDEGTEAEIEKVMNGDYQTSYIEVKRGSKTGGKSAWMLNLSIDVPKIDKGVDPCIIGGIDVGVKSPLVCAINDAFSRYSISDNDLFHFNKKMFARRRILLKKNGHKRAGHGAKNKLKPITIMTEKSKRFRKKLIERWACEIADFFIKNKVGTVQMENLESMKRKEDSYFNIRLRGFWPYAEMQNKIEFKLKQYGIVVRKVAPNNTSKTCSKCGHLNNYFDFEYRRKNKFPHFKCEKCNFKENADYNAALNISNPKLKSTKEEP

SEQ ID NO: 1608 - protein, 726 aa, synthetic construct
SEVEFSHEYWMRHALTLAKRARDEREVPVGAVLVLNNRVIGEGWNRAIGLHDPTAHAEIMALRQGGLVMQNYRLTDATLYVTFEPCVMCAGAMIHSRIGRMVFGVRNSKRGAAGSLMNVLNYPGMNHCVEITEGILVDECAALLCDFYRMPRQVLNAQKKAQSSISSGGSSGGSSGSETPGASGSVTPKSSGGSSAGSTKDTITKTLKLRIVRPYNSAEVEKIVADEKNNREKIALEKNKDKVKEACSKHLKVAAYCTTQVERNACLFCKARKLDDKFYQKLRGQFPDAVFWQELGEIFRQLQKQAAEIYNQSLIELYYEIFIKGKGITNASRVEHYLSDVCYTRAAELFKNAAIASGLRSKVRSNFRLKELKNMKSGLPTTKSDNFPIPLVKQKGGQYTGFEISSHNSDFIIKIPFGRWQEKEEIDKYRPWEKFDFEQVRRSPKPISLLLSTQRRKKNKGWSKDEGTEAEIRKVMNGDYQTSYIEVKRGSKIGEKSAWMLSLSIDVPKIDKGVDPSIIGGIDVGVKSPLVCAINNAFNRYSISDNNLFHFNKKMFARRRILLKKNRHKRAGHGAKNKLKPISILTEKSERFRKKLIERWACEIADFFIRNKVGTVQMENLEGMKRREDSYFNIRLRGFWPYAEMQNKIEFKLKQYGIEVRKVAPNNTSKTCSKCGHLNNYFNFEYRKKNKFPHFKCEKCNFKENADYNAALNISNPKLKSTKEEP

SEQ ID NO: 1609 - protein, 726 aa, synthetic construct
SEVEFSHEYWMRHALTLAKRARDEREVPVGAVLVLNNRVIGEGWNRAIGLHDPTAHAEIMALRQGGLVMQNYRLVDATLYVTFEPCVLCAGAMVHSRIGRVVFGARNSKRGAAGSLMNILNYPGMNHRVEITEGILADECAALLCDFYRMPRQVLSAQKKAQSSVSSGGSSGGSSGSETPGASGSVTPKSSVGSSAGSTKNTITKTLKLRIVRPYNSAEVEKIVADEKNNREKIALEKNRDKVKEACSKHLKVAAYCTTQVERNACLFCKARKLDDKFYQKLRGQFPDAVFWQELGGIFRQLQKQAAEIYNQSLIELYYEIFIKGKGITNASRVEHYLSDVCYTRAAELFKNAAIASGLRGKVKSNFRLKELKSMKSGLPTTKSDNFPIPLVRQKGGQYTGFEISNHNGDFIIKIPFGRWQVKKEICKHRPWEKFDFEQVRKSPKPISLLLSTQRRKRNKGWGKDEGTEAEIRKVMNGDYQTSYIEVKRGSKIGEKSAWMLNLSIDVPKIDKGVDPSIIGGIDVGVKSPLVCAINNAFSRYSISDNDLYRFNKKMFARRRILLKKSKHKRAGHGAKNKLKPITILTEKSGRFRKKLIERWACEIADFFIKNKVGTVQMENLEGMKRKEDSYFNIRLRGFWPYAEMQNKIEFKLKQYGIEIRKVAPNNTSKTCSKCGHLNNYFNFEYRKKNKFPHFKCEKCNFKENADYNAALNISNPKLKSTKEEP

SEQ ID NO: 1610 - protein, 726 aa, synthetic construct
SEVEFSHEYWMRHALTLAKRARDEREVPVGAILVLNNRVIGEGWNRAIGLHDPTAHAEIMALRQGGLVTQNYRLIDATLYVTFEPCVMCAGAMIHSRIGRVVFGVRNSKHGAAGSLMNVLNYPGMNHRVEITEGVLADECAALLSDFYRMPRQVFNAQKKARPYINSGGSSGGSSGSETPGTSESPTPESSGGSSGGSAKNTITKTLKLRIVRPYNSAEVEKIVADEKNNREKIALEKNKDKVKEACSKHLKVAAYCTTQVEGNACLFCKARKLDDKFYQKLRGQFPDAVFWQEIGEIFRQLQKQAAEIYNQSLVELYYEIFIKGKGFANASSVEHYLSDVCYTRAAELFKNAAIASGLRGKVKSNFRLKELKNMKSGLPTTKSDNFPIPLVKQKGGQYTGFEISNHNGDFIIKIPFGRWQVKKEINKHRPWEKFDFEQVRKSPKPISLLLSTQRRKRNKGWSKDEGTEAEIRRVMNGDYQTSYIEVKRGSKIGEKSAWMLNLSIDVPKIDKGVDPSIIGGIDVGVKSPLVCAINNALSRYSISDNDLFHFNKKMFARRRILLRKNRHKRAGHGARNKLKPITVLTEKSERFRKKLIERWACEIANFFIKNKVGTVQMENLESMKRREDSYFNIRLRGFWPYAEMQSKIEFKLKQYGIKIRKVAPNNTSKTCSKCGHLNNYFNFEYRRKNKFPHFKCEKCNFKENADYNAALNISNPKLKSTREEP

SEQ ID NO: 1611 - protein, 726 aa, synthetic construct
SEVEFSHEYWMRHALTLAKRARDEREVPVGAVLVLNNRVIGEGWNRAIGLHDPTAHAEIMALRQGGLVMQNYRLVDATLYVTFEPCVMCAGAMIHSRIGRVVFGVRNNKHGAAGSLVNVLNYPGMNHRVEITEGILADECAALLCDFYRMPRQVFNARKKAQSSINPGGSSGGSSGSETPGTSESATPESSGGSSGSSAKNTITKALKLRIVRPYNSAEVEKIVADEKNNREKIALEKNKDKVKEACSKHLKVAAYCTTQVERNACLFCKARKLDDKFYQKLRGQFPDAVFWQEISEIFRQLQKQAAVIYNQGLIELYYEIFIKGKGIANASRVEHYLSNVCYTRAAELFKNAAIASGLRNKIKSNFRLKELRNMKSGLPTTKSDNFPIPLVKQKGGQYTGFEISSHNSDFIIKIPFGRWQEKEEIDKYRPWEKFDFEQVRRNPKPISLLLSTQRRKRNKGWSKDEGTEAEIRKVMNGDYQTSYIEVKRGSKIGEKSAWMLNLSIDVPKIDKGVDPSITGGIDVGVKSPLVCAINNAFSRYSISDNDLFRFNKKVFARRRILLKKNRHKRAGHGTKNKLKPITILTEKSGRFRKKLIERWACEIANFFIKNKVGTVQMENLESMKRKEDSYFNIRLRGFWPYAEMQNKIEFKLKQYGIKIRKVAPNNTSKTCSKCGHLNNYFSFEYRKKNKFLHFKCEKCNFKEDADYNAALNISNPKLKSTKEEP

SEQ ID NO: 1612 - protein, 726 aa, synthetic construct
SEVEFSHEYWMRHALALAKRARDEREVPVGAILVLNNRVIGEGWNRAISLHDPTAHAEIMALRQGGLVMQNYRLIDATLYVTFEPCVMCAGAMIHSRVGRVVFGVRNSKHGAAGSLMNVLNYPGMNHRVEITEGILADECAALLCDFYRMPRRVFNARRKAQSSTDPGGPSGGSSGSETPGTSESVTPKSSVGSSAGSTKNTITKTLKLRIVRPYNSAEVEKIVADEKNNREKIALEKNKDKVKEACSKHLKVAAYCTTQVERNACLFCKARKLDDKFYQKLRGQFPGAVFWQEIGEIFRQLQKQAAEVYNQSLIELYYEIFVKGKGFANASSVEHYLSDVCYTRAAELFKNAAIASGLRGKVKSNFRLKELRSMRSGLPTTKSDNFPIPLVKQKGGQYTGFEISSHNDDFIIKIPFGRWQVKKEIDKYRPWEKFDFEQVRKSPNPISLLLSTQRRKRNKGWSKDEGTEAEIRKVMNGDYQTSYIEVKRGSKVGEKSAWMLNLSIDVPKIDRGVDPSIIGGIDVGVKSPLVCAINNALNRYSISDNDLFHFNKKMFARRRILLKKNGHKRAGHGAKNKLKPITIMTEKSKRFRKKLIERWACEVADFFIKNRVGTVQMENLESMKRKEDSYFNIRLRGFWPYAEMQNKIEFKLKQYGIVVRKVAPNNTSKTCSKCGHLNNYFNFEYRKKNKFPHFKCEKCNFKEDADYNAALNISNPKLKSTKEEP

SEQ ID NO: 1613 - protein, 726 aa, synthetic construct
SEVEFSHEYWMRHALALAKRARDEREVPVGAVLVLDNRVIGEGWNRAIGLYDPTAHAEIMALRQGGLVMQNYRLTDATLYVTFEPCVMCAGAMIHSRIGRVVFGVRNSKRGAAGSLMNVLNYPGMNHCVEITEGILVDECAALLCDFYRMPRQVLNAQKKAQSSISSGGSSGGSSCSETPGASESVTPKSSGGSSAGSTKNTITKTLKLRIVRPYNSAEVEKIVADEKNSREKIALEKNKDKVREACSKHLKVASYCTTQVERNACPFCKARKLDDKFYQKLRGQFPDAVFWQEIGEIFRQLQKQAAEIYNQSLIELYYEIFIKGKGFANASSVEHYLSDVCYSRAAELFKNAAVASGLRGKVKSNFRLKELKNMKSGLPTTKSDNFPIPLVKQKGGQYTGFEISSHNDDFIIKIPFGRWQVRKEVDKYRPWEKFDFEQVRKSPKPISLLLSTQRRKRNKGWSKDEGTEAEIRKVMNGDYQTSYIEVKRGSKAGEKSAWMLNLSIDVPKIDKGVDPSIIGGIDVGVKSPLVCAINNALSRYSISDNDLFHFNKKMFARRRILLKKNKHKRAGHGARNKLKPITVLTEKSERFRKKLIERWACEIANFFIKNRVGTVQMENLESMRRKEDSYFNIRLRGFWPYAEMQNKIEFKLKQYGIEIRKVAPNNTSKTCSKCGHLNNYFNFEYRKKNKFPHFKCEKCNFKENADYNAALNISNPKLKSTKEEP

SEQ ID NO: 1614 - protein, 726 aa, synthetic construct
SEVEFSHEYWMRHALTLAKRARDEREVPVGAVLVLNNRVIGEGWNRAIGLHDPTAHAEIMALRQGGLVMQNYRLIDATLYVTFEPCVMCAGAMIHSRIGRVVFGVRNNKRGAAGSLMNVLNYPGMNHRVEITEGILADECAALLCDFYRMPRQVLNAQKKARSCINSGGSSGGSSGSETPGTSESATPESSGGSSGGSAKNTITKSLKLRIVRPYNSAEVEKIVADEKDNRERIALEKNKDKVREACSKHLKVASYCTTQVERNACPFCKARKLDDKFYQKLRGQFPDAVFWQELGEILRQLQKQAAEIYNQSLIELYYEIFIKGRGFANASSVEHYLSDVCYTRAAELFKNAAIASGLRGKVKSNFRLKELKNMKSGLPTTKSDNFPIPLVKQKGGQYTGFEISSHNDDFIIKIPFGRWQAKKEIDKYRPWEKFDFEQVRKSPKPISLLLSTQRRKRNRGWSKDEGTEAEIRKVMNGDYQTSYIEVKRGSKIGEKSAWMLSLSIDVPKIDKGVDPSIVGGIDVGVKSPLVCAINNALGRFSISDNDLFHFNKKMFARRRILLRKNRHKRAGHGAKNKLKPISILTEKSKRFRKKLIERWACEIADFFVRNKVGTVQMEDLESMKRRGDSYFNIRLRGLWPYAEMQNKIEFKLKQYGIEIRKVAPNNTSKTCSKCGHLNNYFNFEFRKKNKFPHFKCEKCNFKENADYNAALNISNPKLKSAKEEP

SEQ ID NO: 1615 - protein, 726 aa, synthetic construct
SEVEFSHEYWMRHALTLAKRARDEREVPVGAVLVLNNRVIGEGWNRTTGLHDPTAHAEIMALRQGGLVMRNYRLTDATLYVTFEPCVMCAGAMIHSRIGRVVFGVRNSKRGAAGSLMNVLNYPGMNHCVEITEGILVDECAALLCDFYRMPRQVLNAQKKAQSSISPGGSSGGSSGSETPGASESVTPKSSGGGSSGSAKNTITKTLQLRIVRPYNSAEVEKIVADEKSNREKIALEKNKDKVKEACSKHLKVAAYCTTQVERNACLFCKARKLDDKFYQKLRGQFPDAVFWQEIGEIFRQLQKQAAEIYNQSLIELYYEIFIKGKGFANASSVEHYLSDVCYTRAAELFKNAAIASGLRGKVKSNFRLKELKNMKSGLPTTKSDNFPVPLVKQKGGQYTGFEISSHNDDFIIKIPFGRWQVKEEIDKYRPWEKFDFEQVRKNPKPISLLLSTQRRKRNKGWSKDEGTEAEIRKVMNGDYQTSYIEVKRGSKIGEKSAWMLNLSIDVPKIDKGVDPSIIGGIDVGVKSPLVCAINNAFSRYSISDNDLFRFNKKVFARRRILLKKNRHKRAGHGTKNKLKPITILTEKSGRFRKKLIERWACEIADFFIKNKVGTVQMENLESMKRKEDSYFNVRLRGFWPYAEMQNKIEFKLKQYGIVVRKVAPNNTSKTCSQCGHLNNYFNFEYRKKNQFPYFKCEKCNFKENADYNAALNISNPQLKSTKGEP

SEQ ID NO: 1616 - protein, 726 aa, synthetic construct
SEVEFSHEYWMRHALTLAKRARDEREVPVGAILVLNNRVIGEGWNRAIGLHDPTAHAEIMALRQGGLVMQNYRLTDATLYATFEPCVMCAGAMIHSRIGRVVFGVRNSKHGAAGSLMNVLNYPGMNHRVEITEGILADECAGLLCDFYRMPRQVFSARKKAQSSINPGGSSGGSSGGKAPGTSESATLESSGGSSGSSAKNTITKTLKLRIVRPYNSAEVEKIVADEKNNREKIALEKNKDKVKEACSKHLKVAAYCTTQVERNACLFCKARRLDDKFYQKLRGQFPDAVFWQEIGEIFRQLQKQAAEIYNQSLIELYYEIFIKGKGFANASSVEHYLSDVCYTRAAGLFKNAAIASGLRGKVKSNFRLKELKNMKSGLPTTKSDNFPIPLVKQKGGQYTGFEISSHNDDFIIKIPFGRWQVKKEIDKYRPWEKFDFEQVRKCPKPISLLLSTQRRKRNKGWSKDEGTEAEIRKVMNGDYQTSYIEVKRGSKIGEKSAWMLNLSIDVPKIDKGVDPSIIGGIDVGVKSPLVCAINNALSRYSISDNDLFHFNKKMFARRRILLRKNRHKRAGHGARNKLKPITVLTEKSERFRKKLIERWACEIANFFIKNKVGTVQMENLESMKRREDSYFNIRLRGFWPYAEMQNKIEFKLKQYGIEIRKVAPNNTSKTCSKCGHLNNYFSFEFRKKNKFPRFKCEKCSFKENADYNAALNISNPKLKSTKGEP

SEQ ID NO: 1617 - protein, 726 aa, synthetic construct
SEVEFSHEYWMRHALTLAKRARDEREVPVGAVLVLNNRVIGEGWNRAIGLHDPTAHAEVMALRQGGLVMQNYRLTDATLYVTFEPCVMCAGAMIHSRIGRVVFGVRNSKRGAAGSLMNVLDYPGMNHCVEITEGILVDECAALLCDFYRMPRQVLNAQKKAQSSISSGGSSGGSSGSVTPGASGSVTPKSSGGSSAGSTKDTITKTLKLRIVRPYNSAEVEKIVADEKNSREKIALEKYKDKVKEACSEHLKVAAYCTTQVERNACLFCKARKLDDRFYQKLRGQFPGAVFWQEIGEIFRQLQKQAAEIYNQSLIELYYEIFIKGKGFANASSVEHYLSDVCYTRAAELFKNAAIASGLRGKVKSNFRLKELKNMKSGLPTTKSDNFPIPLVKQKGGQYTGFEINSHNDDFIIKIPFGRWQVKKEIDKYRPWEKFDFEQVRKGPKPISLLLSTRRRKRNKGWSKDEGTEAEIRKVMNGDYQTSYIEVKRGSKIGEKSAWMLNLSIDVPKIDKGVDPSIIGGIDVGVKSPLVCAINNSSSRYSICDNDLFRFNKKMFARRRILLKKNRHKRAGHGAKNKLKPITILTKKSERFRKKLIERWVCEVADFFIKNKVGTVQMENLESMKRKEDSYFNIRLRGFWPYAEMQNRIELKLKQYGIEIRRVAPNNTSKTCSKCGHLNSYFNFEYRKKNKFPHFKCEKCNFKEDADYNAALNISNPKLKSTKEEP

SEQ ID NO: 1618 - protein, 726 aa, synthetic construct
SEVEFSHEYWMRHALTLARRARDEREVPVGAVLVLNNRVIGEGWNRAIGLHDPTAHAEIMALRQGGLVMQNYRLTDATLYVTFEPCVMCAGAMIHSRIGRVVFGVRNSKRGAAGSLMNVLSYPGMNHCVEITEGILVDECAALLCDFYRMPRQVLNAQKKAQSSISSGGSSGGSSGSETPGASESVTPKSSVGSSASSTKNTITKTLKLRIVRPYNSAEVEKIVADEKNNREKTALEKNKGKVKEACSKHLKVATYCTTQVERNACLFCKARKLDDKFYQKLRGQFPDAVFWQEIGEIFRQLQKQAAEIYNQSLIELYYEIFIEGKGSANARSVEHYLSDVCYTRAAELFKNAAIASGLRGKVKGNFRLKELKNMKSGLPTTKSDNFPIPLVKQKGGQYTGFEISSHNDDFIIKIPFGRWQVRKEIDKYRPWEKYNFEQVRKSPKPISLLLSTQRRKRNKGWSKDEGTEAEIRKVMNGDYQTSYIEVKRGSKIGEKSAWVLNLSIDVPKIDRGVDPSIIGGIDVGVKSPLVCAINNAFSRYSISDNDLFRFNKKVFARRRILLKKNRHKRAGHGTKNKLKPITILAEKSGRFRKKLIERWACEIANFFIKNKVGTVQMENLESMKRKEDSYFNIRLRGFWPYAEMQNKIEFKLKQYGIKIRKVAPNNTSRTCSECGHLNNYFSFEYRKKNKFPHFKCEKCNFKEDADYNAALNISNPKLKGTKEEL

SEQ ID NO: 1619 - protein, 726 aa, synthetic construct
SEVEFSHEYWMRHALTLAKRARDEREVPVGAILVLNNRVIGEGWNRAIGLHDPTAHAEIMALRQGGLVMQNYRLIDATLYVTFEPCVMCAGAMIHSRIGRVVFGVRNSKHGAAGSLMNVLNYPGMNHRVEITEGILADECAALLCDFYRMPRQVFNARKKAQTSISSGGSSGGSSGSETPGANGSVTPKSSGGSTAGSTKDTITKTLKLRIVRPYNSAEVEKVVADEKNNREKIAMEKNKDKVKEACSKHLKVASYCTTQVERNACLFCKARKLDDKFYQKLRGQFPDAVSWQELGGIFRQLQKQAAEIYNQSLIELYYEIFIKGKGITSASRVEHYLSDVCYTRAAELFKNAAIASGLRSKVRSNFRLKELKNMKSGLPTTKSDNFPIPLVKQKGGQYTGFEISSHNDDFIIKIPFGRWQVKKEIDKYRPWEKFDFEQVRKSPKPISLLLSTQRRKRNKGWSKDEGTEAEIRKVMNGDYQTSYIEVKRGSKIGEKSAWMLNLSIDVPKTDKGVDPSIIGGIDVGVRSPLVCAINNAFSRYSISDNDLFHFNKKMFARRRILLRKNRHKRAGHGARNKLKPITVLTEKSERFRKKLIERWACEIANFFIKNKVGTVQMENLESMKRKEDSYFNIRLRGFWPYAEMQNKIEFKLKQYGIEIRKVAPNNTSKTCSRCGHLNNYFNFEYRKKNKFPHFKCEKCNFKEDADYNAALNISNPKLKSTKEEP

SEQ ID NO: 1620 - protein, 726 aa, synthetic construct
SEVEFSHEYWMRHALTLAKRARDEREVPVGAILVLNNRVIGEGWNRAIGLHDPTAHAEIMALRQGGLVMQNYRLTDATLYATFEPCVMCAGAMIHSRIGRVVFGVRNNRHGAAGSLMNVLNYPGMNHRVEITEGILADECAGLLCDFYRMPRQVFSARKKAQSSISSGGSSGGSSGSETPGASESVTPKSSGGSSAGSTKNTITKTLKLRIVRPYNSAEVEKIVADEKNNREKIALEKNKDKVKEACSKHLKVAAYCTTQVERNACLFCKARRLDDKFYQKLRGQFPDAVFWQEIGEIFRQLQKQAAEIYNQSLIELYYEIFIKGKGFANASSVEHYLSDVCYARAAELFKNAAIASGLRGKVKSNFRLKELKNMKSGLPTTKSDNFPIPLVRQKGGQYTGFEISSHNDDFIIKIPFGRWQVKKEIDKYRPWEKFDFEQVRKSPKPISLLLSTQRRKRNKGWSKDEGTEAEIRKVMNGDYQTSYIEVKRGSKTGEKSAWMLNLSIDVPKIDKGVDPSIIGGIDVGVKSPLVCAINNAFSRYSISDNDLFHFNKKMFARRRILLRKNRHKRAGHGARNKLKPITVLTEKSKRFRKKLIERWACEIADFFIKNKVGTVQMENLESMKRKEDSYFNIRLRGFWPYAEMQNKIEFKLKQYGIKIRKVAPNNTSRTCSKCGHLNNYFSFEYRKKNKFPHFKCEKCNFKEDADYNAALNISNPKLKGTKEEL

SEQ ID NO: 1621 - protein, 726 aa, synthetic construct
SEVEFSHEYWMRHALTLAKRARDEREVPVGAVLVLNNRVIGEGWNRAIGLHDPTAHAEIMALRQGGLVMQNYRLTDATLYVTFEPCIMCAGAMIHSRIGRVVFGVRNSKRGAAGSLMNVLNYPGMNHRVEITEGILADECTALLCDYYRMPRQVFNARKKVQSSINSGGSSDGGSGSETPGASGSVTPKSSVGSPAGSTKNTITKTLKLRIVRPYNSAEVEKIVADEKNNREKIALEKNKDKVKEACSKHLEVAAYCTTQVERNACLFCKARKLDDKFYQKLRGQFPDAVFWQEIGEIFRQLQKQAAEIYNQSLIELYYEIFIKGKGFANASSVEHYLSDVCYTRAAELFKNAAIASGLRNKTKSNFRLKELRSMKSGLPTTKSDNFPIPLVKQKGGQYTGFEISNHNSDFIIKIPFGRWQAKKEIDKYRPWEKFDFEQVRKSPKPISLLLSTQRRKRNKGWSKDEGTEAEIEKVMNGDYQTSYIEVKRGSKTGGKSAWMLNLSIDVPKIDKGVDPCIIGGIDVGVKSPLVCAINDAFSRYSISDNDLFHFNKKMFARRRILLKKNGHKRAGHGAKNKLKPITIMTEKSKRFRKKLIERWACEIADFFIKNKVGTVQMENLESMKRKEDSYFNIRLRGFWPYAEMQNKIEFKLKQYGIEIRKVAPNNTSKTCSKCGHLNNYFSFEYRKKNKFPHFKCEKCNFKEDADYNAALNISNPKLKSTKEEP

SEQ ID NO: 1622 - protein, 726 aa, synthetic construct
SEVEFSHEYWMRHALALAKRARDAREVPVGAILVLNNRVIGEGWNRAIGQHDPTAHAEIMALRQGGLVMQNYRLIDATLYVTFEPCVMCAGAMIHSRIGRVVFGVRNSKHGAAGSLMNVLNYPGMNHRVEITEGILADECAALLCDFYRMPRQVFNGRKKAQSSINSGGSSGGSSGSEAPGTSESATPESSGGSSGGSAKNTITKTLQLRIVRPYNSAEVEKIVADEKNNREKIALEKNKDKVKEACSKHLKVAAYCTTQVERNACLFCKARKLDDKFYQKLRGQFPDAVFWQETGEIFRQLQRQAAEIYNQSLIELYYEIFIKGKGFANASSVEHYLSDVCYTRAAELFKNAAIASGLRGKVKGNFRLKELKNMKSGLPTTKSDNFPIPLVRQKGGQYTGFEISSHNDDFIIKIPFGRWQAKKEIDKYRPWEKFDFEQVRKSPKPISLLLSTQRRKRNKGWSKDEGTEAEIRKVMNGDYQTSYIEVKRGSKIGEKSAWMLNLSIDVPKIDKGVDPSIIGGIDVGVKSPLVCAINNAFSRYSISDNDLFHFNKKMFARRRILLKKNRHKRAGHGAKNKLKPISILTEKSKRFRKKLIERWACEIADFFIKNKVGTVQMENLESMKRKEDSYFNIRLRGFWPYAEMQNKIEFKLKQYGIEIRKVAPNNTSKTCSKCGHLNNYFNFEYRRKNKFPYFKCEKCNFKENADYNAALNISNPQLKSTKGEP

SEQ ID NO: 1623 - protein, 726 aa, synthetic construct
SEVEFSHEYWMRHALSLAKRARDEREVPVGAVLVLNNRIIGEGWNRAIGLHDPTAHAEIMALRQGGLVMQNYRLTDATLYVTFEPCVMCAGAMVHSRIGRVVFGVRNSKRGAAGSLMNVLNYPGVNHCVEITEGILVDECAALLCDFYRMPRQVLNAQKKAQSSISSGGSSGGCSGSETPGTSESPTPESSGGSPGGSAKNTITKTLKLRIVRPYNSAEVEKIVADEKNNREKIALEKNKDKVKEACSKHLKVAAYCTTQVERNACLFCKARKLDDKFYQKLRGQFPDAVFWQEIGEIFRQLQKQAAEIYNQSLIELYYEIFIKGKGFANASSVEHYLSDVCYTRAAELFKNAAIASGLRGKVKSNFRLKELKNMKSGLPTTKSDNFPIPLVKQKGGQYTGFEISSHNSDFIIKIPFGRWQVKEEIDKYRPWEKFDFEQVRKSPKPISLLLSTQRRKKNKGWSKDEGTEAEIRRVMNGDYQTSYIEVKRGSKIGEKSAWMLNLSIDVPKIDKGVDPSIIGGIDVGVKSPLVCAINNSSSRYSICDNDLFRFNKKMFARRRILLKKNRHKRAGHGAKNKLKPITILTKKSERFRKKLIERWVCEVADFFVKNKVGTVQMENLEGMKRKEDSYFNIRLRGFWPYAEMQNKIEFKLKQYGIEIRKVAPNNTSKTCSKCGHLNDYFNFEYRKKNKFPHFKCEKCNFKENADYNAALNISNPKLKSTKEEP

SEQ ID NO: 1624 - protein, 726 aa, synthetic construct
SEVEFSHEYWMRHALTLAKRARDEREVPVGAVLVLNNRAIGEGWNRAIGLHDPTAHAEIMALRQGGLVMQNYRLTDATLYVTFEPCVMCAGAMIHSRIGRVVFGVRNSKRGAAGSLMNVLNYPGMNHCVEITEGILVDECAALLCDFYRMPRQVLNAQKKAQSSISSGGSSGGSSGSETPGASGSVIPKSSGGSSAGSTKDTITKTLKLRIVRPYNSAEVEKVVADEKNNREKIALEKNKDKVKEACSKHLKVASYCTTQVERNACPFCKARKLDDKFYQKLRGQFPDAVFWQELGEILRQLQKQAAEIYNQSLIELYYEIFIKGKGIANASSVEHYLSDVCYTRAAELFKNAAIASGLRNKIKSNFRLKELRNMKSGLPTTKSDNFPIPLVRQKGGQYTGFEISNHDGDFIIKIPFGRWQVKKEINKHRPWEKFDFEQVRKSPKPISLLLSTQRRKRNKGWSKDEGTEAEIRKVMNGDYQTSYIEVKRGSKIGEKSAWMLNLSIDVPKIDKGVDPGIIGGIDVGVKSPLVCAINNASSRYSISDNDLFHFNKKMFARRRILLRKNRHKRAGHGARNKLKPITVLTEKSERFRKKLIERWACEIANFFIKNKVGTVQMENLESMKRREDSYFNIRLRGFWPYAEMQSKIEFKLKQYGIKIRKVAPNNTSKTCSKCGHLNNYFNFEFRKKNKFPHFKCEKCNFKEDADYNAALNISNPKLKSTKEEP

SEQ ID NO: 1625 - protein, 726 aa, synthetic construct
SEVEFSHEYWMRHALTLAKRARDEREVPVGAVLVLNNRVIGVGWNRAIGLHDPTAHAEIMALRQGGLVMQDYRLTDATLYVTFEPCVMCAGAMVHSRIGRVVFGVRNSKRGAAGSLMNVLNYPGMSHCVEITEGILVDECAALLCDFYRMPRQVLNAQKKAQSSISSGGSSGGSGGGETPGASESVTPESSGGGSSGSAKNTITKTLQLRIVRPYNSAEVEKIVADEKNNREKIALEKNKDKVKEACSEHLKVAAYCTTQVERSACLFCKARKLDDKFYQKLRGQFPDAVFWQEIGEIFRQLQKQAAEIYNQSLIELYYEIFIKGKGITNASRVEHYLSDVCYTRAAELFKNAAIASGLRSKVRSNFRLKELKNMKSGLPTTKSDNFPIPLVKQKGGQYTGFEISSHNDDFIIKIPFGRWQVKKEIVKYRPWEKFDFEQVRKSPKPISLLLSTQRRKRNKGWSKDEGTEAEIRKVMNGDYRTSYIEVKRGSKTGEKSAWMLNLSIDVPKIDKGVDPSIIGGIDVGVKSPLVCAINNAFSRYSISDNDLFRFNKKMFARRRILLKKNRHKRAGHGARNKLKPITVLTEKSERFRKKLIERWACEIAYFFIKNKVGTVQMENLESMKRKEDSYFNTRLRGFWPYAEMQNKIEFKLKQYGIEIRKVAPNNTSKTCSKCGHLNNYFNFEYRKKNKFPPFKCEKCDFKENADYNAALNISNPELKGAKEEP

SEQ ID NO: 1626 - protein, 726 aa, synthetic construct
SEVEFSHEYWMRHALTLAKRARDEREVPVGAVLVLNNRVIGEGWNCTTGLHDPTAHAEIMALRQGGLVMQNYRLIGATLYVTFEPCAMCAGAMIHSRIGRVVFGVRNSKRGAAGSLMNVLNYPGMNHRVEIMEGILTDECAALLCDFYRMPHQVLNAQKKAQSSINPGGSSGDSSGGKAPGTSESATLESSGGSSGDSAKNSITKTLKLRIVRPYNSAEVEKIVADEKNNREKIAMEKNKDKVKEACSKHLKVASYCTTQVERNACLFCKARKLDDKFYQKLRGQFPDAVFWQELGGIFRQLQKQAAEIYNQSLIELYYEIFIKGKGITNASRVEHYLSDVCYTRAAELFKNAAIASGLRSKVRSNFRLKELKNMKSGLPTTKSDNFPIPLVKQKGGQYTGFEISSHNSDFIIKIPFGRWQEKEEIDKYRPWEKFDFEQVRKSPKPISLLLSTQRRKRNKGWSKDEGTEAEIRRVMNGDYQTSYIEVKRGSKIGEKSAWMLNLSIDVPKIDKGVDPSIIGGIDVGVKSPLVCAINNSSSRYSICDNDLFRFNKKMFARRRILLKKNRHKRAGHGAKNKLKPITILTKKSERFRKKLIERWVCEVADFFIKNKVGTVQMENLESMKRKEDSYFNVRLRGFWPYAEMQNKIEFKLKQYGIVVRKVAPNNTSKTCSKCGHLNNYFSFEYRKKNKFPHFKCEKCNFKEDADYNAALNISNPKLKSTKGEP

SEQ ID NO: 1627 - protein, 726 aa, synthetic construct
SEVEFSHEYWMRHALTLAKRARDEREVPVGAVLVLNNRVIGEGWNRAIGLHDPTAHAEIMALRQGGLVMQNYRLSDATLYVTFEPCVMCAGAMIHSRIGRVVFGVRNSKRGAAGSLMNVLNYPGMDHCVEITEGILVDECAALLCDFYRMPRQVLSAQKKAQSSVSSGDSSGGSSGSETPGASGSVTPKSSVGSSAGSTKNTITKTLKLRIVRPYNSAEVEKIVADEKNNREKIALEKNRDKVKEACSKHLKVAAYCTTQVERNACLFCKARRLDDKFYQKLRGQFPDAVFWQEIGEIFRQLQKQAAEIYNQSLVELYYEIFIKGKGIANASSVEHYLSDVCYTRAAELFKNAAIASGLRNKIKSNFRLKELKNMKSGLPTTKSDNFPIPLVRQKGGQYTGFEISSHNDDFIIKIPFGRWQVRKEIDKYRPWEKFDFEQVRKSPKPISLLLSTQRRKRNKGWSKDEGTEAEIRKVMNGDYQTSYIEVKRGSKTGEKSAWMLNLSIDVPKIDKGVDPSIIGGIDVGVKSPLVCAINNALSRYSISDNDLFHFNKKMFARRRILLRKNRHKRAGHGARNKLKPITVLTEKSERFRKKLIERWACEIANFFIKNKVGTVQMENLESMKRREDSYFNIRLRGFWPYAEMQNKIEFKLKQYGIEIRKVAPNNTSKTCSKCGHLNNYFNFEYRKKNKFPHFKCEKCNFKENADYNAALNISNPKLKSTKEEP

SEQ ID NO: 1628 - protein, 726 aa, synthetic construct
SEVEFSHEYWMRHALTLAKRARDEREVPVGAVLVLNNRVIGEGWNRAIGLHDPTAHAEIMALRQGGLVMQNYRLIDATLYVTFEPCVMCAGAMIHSRIGRVVFGVRNNKHGAAGSLVNVLNYPGMNHRVEITEGILADECAALLCDFYRMPRQVFNARKKAQSSINSGGSSGGSSGSETPGTSESATPKSSGGSSGGSAKNTITKTLTLRIVRPYNSAEVEKIVADEKNNREKIALEKNKDKVKEACSEHLKVAAYCTTQVGRNACLFCKARKLDDKFYQKLRGQFPDAVFWQEIGEIFRQLQKQAAEVYNQSLIELYYEIFIKGKGFANASSVEHYLSDVCYARAAELFKNAAIASGLRGKVKSNFRLKELKNMKSGLPTTKSDNFPIPLVKQKGGQYTGFEISSRNDDFIIKIPFGRWQGKKEVDKYRPWEKFDFEQVRKSPKPISLLLSTQRRKRNKGWSKDEGTEAEIKKVMNGDYQTSYIEVKRGSKIGEKSAWMLSLSIDVPKIDRGVDPSIIGGIDVGVKSPLVCAINNASSRLSISDNDLFRFNKKMFARRRILLKKNGHKRAGHGAKNKLKPITILTEKSVRFRKKLIERWACEIADFFIRNKVGTVQMENLESMKRKEDSYFNIRLRGFWPYAEMQNKIEFKLKQYGIEIRKVAPNNTSKTCSKCGHLNNYFNFEYRKKNKFPHFKCEECNFKENADYNAALNISNPKLKSTKEEP

SEQ ID NO: 1629 - protein, 726 aa, synthetic construct
SEVEFSHEYWMRHALTLAKRARDEREVPVGAVLVLNNRVIGEGWNRAIGLHDPTAHAEIMALRQGGLVMRNYRLTDATLYVTFEPCVMCAGAMIHSRIGRVVFGVRNSKRGAAGSLMNVLNYPGMNHRVEITEGILADECAALLCDFYRMPRQVFNARKKAQSSINPGGSSGGSSGSETPGASESATPESSGGSSGGSAKNTITKTLKLRIVRPYNSAEVEKIVADEKNNREKIALEKNKDKVKEACGKHLKVAAYCTTQVERNACLFCKARRLDDKFYQKLRGQFPDAVFWQEVGEIFRQLQKQAAEIYNQSLIELYYEIFIKGKGFANASSVEHYLSDVCYTRAAELFKNAAIASGLRGKVKSNFRLKELKNMKSGLPTTKSDNFPIPLVKQKGGQYTGFEISSHNDDFIIKIPFGRWQVKEEIDKYRPWEKFDFEQVRKNPKPISLLLSIQRRKRNKGWSRDEGTEAEIRKVMNGVYQTSYIEVKRGSKIGEKSAWMLNLSIDVPRIDKGVDPSIIGGIDVGVKSPLICAINNAFSRYGISDNDLFRFNKKVFARRRILLKKNRHKRAGHGTKNKLKPITILTEKSGRFRKKLIERWACEIANFFIKNKVGTVQMEDLESMKRKEDSYFNIRLRGFWPYAEMQNKIEFKLKQYGIKIRKVAPNNTSKTCSKCGHLNNYFNFEYRKKNKFPHFKCEKCNFKEDADYNAALNISNPKLKSTKEEP

SEQ ID NO: 1630 - protein, 726 aa, synthetic construct
SEVEFSHEYWMRHALTLAKRARDEREVPVGAVLVLNNRVIGEGWNRAIGLHDPTAHAEIMALHQGGLVMQNYRLIDATLYVTFEPCVMCAGAMIHSRIGRVVFGARNSKRGAAGSLMNVLSYPGMNHRVEITEGILADECAALLCDFYRMPRRVFNAQKKAQSSINSGGSSGGGSGSETPSTSESTTPESSGGSSGGPAKNTITKTLKLRIVRPYNSAEVEKIVADEKNNREKIALEKNKDKVKEACSKHLKVAAYCTTQVERDACLFCKARKLDDKFYQKLRGQFPDAVFWQELGEILRQLQKQAAEIYNQSLIELYYEIFIKGRGFANASSVEHYLSDVCYTRAAELFKNAAIASGLRGKVKSNFRLKELKNMKSGLPTTKSDNFPIPLVKQKGGQYTGFEISSHNDDFIIKIPFGRWQVRKEIDKYRPWEKFNFEQVRKSPKPISLLLSTQRRKRNKGWSKDEGTEAEIRKVMNGDYQTSYIEVKRGSKIGEKSAWMLNLSIDVPKIDEGVDPSIIGGIDVGVKSPLVCAINNAFSRYSISDNDLFRFNKKVFARRRILLKKNRHKRAGHGTKNKLKPITILTEKSGRFRKKLIERWACEIANFFIKNKVGTVQMENLESMKRKEDSYFNIRLRGFWPYAEMQNKIEFKLKQYGIKIRKVAPNNTSKTCSKCGHLNNYFSFEYRKKNKFPHFKCEKCNFKEDADYNAALNISNPKLKSTKEEP

SEQ ID NO: 1631 - protein, 726 aa, synthetic construct
SEVEFSHEYWMRHALTLAKRARDEREVPVGAILVLNNRVIGEGWNRAIGLHDPTAHAEIMALRQGGLVMQNYRLIDATLYVTFEPCVMCAGAMIHSRIGRVVFGVRNNKHGAAGSLVNVLNYPGMNHRVEITEGILADECAALMCDFYRMPRQVFNARKKAQSSTNPGGSSGGSSGSETPGTSESATPESPGGSSSGSAKNTITKTLQLRIVRPYNSAEVEKIVADEKNNREKIALEKNKDKVKEACSKHLKVAAYCTTQVERNACLFCKARKLDDKFYQKLRGQFPDAVFWQEIGEIFRQLQKQAAEIYNQSLIELYYEIFIKGKGFANASSVEHYLSDVCYTRAAELFKNAAIASGLRGKVKSNFRLKELKNMRSGLPTTKSDNFPIPLVKQKGGQYTGFEISSYNDDLIIKIPFGRWQVKKEIDKYRPWEKFDFEQVRKSPKPISLLLSTQRRKRNKGWSKDEGTEAEIRKVMNGDYQTSYIEVKRGSKIGEKSAWMLNLSIDVPKIDKGVDPSIIGGIDVGVKSPLVCAINNAFSRYSISDNELFHFNKKMFARRRILLKKNRHKRAGHGAKNKLKPISVLTEKSGRFRKKLIERWACEIANFFIKNKVGAVQMENLESMKRREDSYFNIRLRGFWPYAEMQNKIEFKLKQYGIEIRKVAPNNTSKTCSKCGHLNNYFNFEFRKKNKFPHFKCEKCNFKENADYNAALNISNPKLKSTKEEP

SEQ ID NO: 1632 - protein, 726 aa, synthetic construct
SEVEFSHEYWMRHALTLAKRARDEREVPVGAVLVLNNRVIGVGWNRAVGLHDPTAHAEIMALRQGGLVMQNYRLIEATLYVTFEPCIMCAGAMIHSRIGRVVFGVRNSKRGAAGSLMNVLNYPGMNHRVEITEGILADECAALICDYYRMPRQVFNARKKAQPSINSGGSSDGGSGSETPGTSESATPESSGSSSGGSAKNTITKTLKLRIVRPYNSAEVEKIVADEKNNRERIALEKNKDKVKEACSKHLKVAAYCTTQVERNACLFCKARKLDDKFYQKLRGQFPDAVFWQEIGEIFRQLQKQAAEIYNQSLIELYYEILIKGKGFANASSVEHYLSDVCYTRAAELFKNAAIASGLRGKVKSNFRLRELKSMKSGLPTTKSDNFPIPLVKQKGGQYTGFEISSHNDDFIIKIPFGRWQAKKEIDKYRPWEKFDFEQVRKSPKPISLLLSTQRRKRNRGWSKDEGTEAEIRKVMNGDYQTSYIEVKRGSKIGEKSAWMLNLSIDVPKIDKGVDPSIIGGIDVGVKSPLVCAINNAFSRYSISDNDLFRFNKKMFARRRILLGKNRHKRAGHGVKNKLKPITILTEKSGRFRKKLIERWACEIADFFVKNKVGTVQMENLESMKRKEDSYFNIRLRGFWPYAEMQNKIEFKLKQYGIKVRKVAPNNTSKTCSKCGHLNNYFSFEYRKKNKFPHFKCEKCNFKENADYNAALNISNPKLKSTKEEP

SEQ ID NO: 1633 - protein, 726 aa, synthetic construct
SEVEFSHEYWMRHALTLAKRARDEREVPVGAVLVLNNRVIGEGWNRAIGLHDPTAHAEIMALRQGGLAMQNYRLVDATLYVTFEPCVLCAGAMVHSRIGRVVFGVRNSKRGAAGSLMNVLNYPGMNHRVEITEGILADECAALLCDFYRMPRQVFNARKKARSNINSGGSSGGSSGSETPSTSESATPESSGGSSGGSARNTITKTLQLRIVRPYNSAEVEKIVTDEKNNREKIALEKNKDKVKEACSKHLKMASYCTTQVERNACLFCKARKLDDKFYQKLRGQFPDAVFWQELGGIFRQLQKQAAEIYNQSLIELYYEIFIKGKGFTNASRVEHYLSDVCYTRAAELFKNAAIASGLRSKVRSNFRLKELKNMKSGLPTTKSDNFPIPLVKQKGGQYTGFEISSHNSDFIIKIPFGRWQVKEEIDKYRPWEKFDFEQVRKSPKPISLLLSTQRRKRNKGWSKDEGTEAEIRKVMNGDYQTSYIEVKRGSKIGEKSAWMLNLSIDVPKIDKGVDPSIIGGIDVGVKSPLVCAINNAFSRYSISDNDLFHFNKKVFARRRILLKKNRHKRAGHGVKNKLKSISILTEKSKRFRKKLIERWACEIADFFIKNKVGTVQMENLESMKRKEDSYFNIRLRGFWPYAEMQNKIEFKLKQYGIEIRKVAPNNTSKTCSKCGHLNNYFNFEYRRKNKFPHFKCEKCNFKEDADYNAALNISNPKLKSTKEEP

SEQ ID NO: 1634 - protein, 726 aa, synthetic construct
SEVEFSHEYWMRHALTLAKRARDEREVPVGAVLVLNNRVIGEGWNRAIGLHDPTAHAEIMALRQGGLVMQNYRLTDATLYVTFEPCVMCAGAMIHSRIGRVVFGVRNSKHGAAGSLVNVLNYPGMNHRVEITEGILADECAALLCDFYRMPRQVLNAQKKAQSSISSGGSSGGSSGSETPGASESATPKSPGGSSASSIKNTITKTLKLRIVRPYNSAEVEKIVADEKNNRERIALEKNKDKVKEACSKHLKVAAYCTTQVERNACLFCKARKLDDKFYQKLRGQFPDAVFWQELGEIFRQLQKQAAEIYNQGLIELYYEIFIKGKGVANANNVEHYLSDVCYTRAAELFKNAAIASGLRNKIKSNFRLKELRNMKSGLPTTRSDNFPIPLVKQKGGQYTGFEISSHNSDFIIKIPFGRWQVKEEIDKYRPWEKFDFEQVRKSPKPISLLLSTQRRKKNKGWSKDEGTEAEIRRVMNGDYQTSYIEVKRGSKIGEKSAWMLNLSIDVPKIDKGVDPSIIGGIDVGVKSPLVCAINNSSSRYSICDNDLFRFNKKMFARRRILLKKNRHKRAGHGAKNKLKPITILTKKSERFRKKLIERWVCEVADFFIKNKVGTVQMENLESMKRKEDSYFNIRLRGFWPYAEMQNRIELKLKQYGIEIRRVAPNNTSRTCSKCGHLNNYFNFEYRKKSKFPHFKCEKCNFREDADYNAALNISNPKLKSTKEEP

SEQ ID NO: 1635 - protein, 726 aa, synthetic construct
SEVEFSHEYWMRHALTLAKRARDEREVPVGAILVLNNRVIGVGWNRAIGLHDPTAHAEIMALRQGGLVTQNYRLIDATLYVTFEPCVMCAGAMIHSRIGRVVFGVRNSKHGAAGSLVNVLNCPGMNHRVEITEGILADECAALLCDFYRMPRQVFNAQKKARPNINSGGSSGGRSGSETPGTSESATPESSGGSSGGSAKNTITKTLKLRIVRPYNSAEVEKIVADEKNSREKIALEKNKDKVKEACSEHLKVAAYCTTQVERNACLFCKARKLDDKFYQKLRGQFPDAVFWQEIGEIFRQLQRQAAEIYNQSLIELYYEIFIKGKGFANASSVEHYLSDVCYTRAAELFKNAAIASGLRGKVKSNFRLKELKNMKSGLPTTKSDNFPIPLVKQKGGQYTGFEVSSHNDDFIIKIPFGRWQVKKEIDKYRPWEKFDFEQVRKSPKPISLLLSTQRRKRNKGWSKDVGTEAEIRKVMNGDYQTSYIEVKRGSKIGEKSAWMLSLSIDVPKIDKGVDPSIIGGIDVGVKSPLVCAISNAFSRYSISDNDLFHFNKKMFARRRILLKKSKHKRAGHGAKNKLKPITILTEKSRRFRKKLIERWACEIADFFIKNKVGTVQMENLESMKRREDSYFNIRLRGFWPYAEMQNKIEFKLKQYGIEIRKVAPNNTSKTCSKCGHLNNYFSFEYRKKNKFPHFKCEKCNFKENADYNAALNISNPKLMSTKEGP

SEQ ID NO: 1636 - protein, 726 aa, synthetic construct
SEVEFSHEYWMRHALTLAKRARDEREVPVGAVLVLNNRVIGEGWNRAIGLHDPTAHAEIMALRQGGLVMQNYRLTDATLYVTFEPCVMCAGAMIHSRIGRVVFGVRNSKRGAAGSLMNVLNYPDMNHCVEITEGILVDECAALLCDFYRMPRQVLNAQKKAQSSISSGGSSGGSSGSETPGASESATPKSSGGSSAGSTKNTITKTLKLRIVRPYNSAEVEKIVADEKNNRERIALEKNKDKVKEACSKHLKVAAYCTTQVERNACLFCKARKLDDKFYQKLRGQFPDAVFWQELGEIFRQLQRQAAEIYNQSLIELYYEIFIKGKGFANASSVEHYLSDVCYTRAAELFKNAAIASGLRSKVRGNFRLKELKNMKSGLPTTKSDNFPIPLVKQKGGQYTGFEISSHNSDFIIKIPFGRWQVKEEIDKYRPWEKFDFEQVRKSPKPISLLLSTQRRKKNKGWSKDEGTEAEIRRVMNGDYQTSYIEVKRGSKIGEKSAWMLNLSIDVPKIDKGVDPSIIGGIDVGVKSPLVCAINNSFSRYSICDNDLFRFNKKMFARRRILLKKNRHKRAGHGAKNKLKPITILTKKSERFRKKLIERWVCEVADFFIKNKVGTVQMENLESMKRKEDSYFNIRLRGFWPYAEMQNRIELKLKQYGIEIRRVAPNNTSRTCSKCGHLNNYFNFEYRKKNKFPHFKCEKCNFREDADYNAALNISNPKLKSTKEEP

SEQ ID NO: 1637 - protein, 726 aa, synthetic construct
SEVEFSHEYWMRHALTLAKRARDEREVPVGAVLVLNNRVIGEGWNRAIGLHDPTAHAEIMALRQGALVMQNYRLTDATLYVTFEPCVMCAGAMIHSRIGRVVFGVRNSKRGAAGSLMNVLNYPGMNHCVEITEGILMDECAALLCDFYRMPRQVLNAQKKAQSSISSGGPSGSSSCSETPGASESVTPKSSGGSSTGSTKNTITKTLKLRIVRPYNSAEVEKIVADEKNSREKIALEKNKDKVKEACSEHLKVAAYCTTQVERNACLFCKARKLDDRFYQKLRGQFPDAVFWQEIGEIFRQLQKQAAGIYNQSLIELYYEIFIKGRGFANASSVEHYLSDVCYTRAAELFKNAAIASGLRGKVKGNFRLKELKNMKSGLPTTKSDNFPIPLVKQKGGQYTGFEISSHNDDFIIKIPFGRWQVKKEIDRYRPWEKFDFEQVRKSPKPISLLLSTQRRKRNKGWSKDEGTEAEIRKVMSGDYQTSYIEVKRGSKTGEKSAWMLNLSIDVPKIDKGVDPSIIGGIDVGVKSPLVCAINNAFSRYSISDNDLFRFNKKMFARRRILLKKNRHKRAGHGAKNKLKPISILTGKSERFRKKLIERWACEIADFFIKNKVGTVQMENLESMKRREDSYFNIRLRGFWPYAEMQNKIEFKLKQYGIEIRKVAPNNTSKTCSKCGHLNNYFNFEYRKKNKFPHFKCEKCNFKENADYNAALNISNPKLKSTKEEP

SEQ ID NO: 1638 - protein, 726 aa, synthetic construct
SEIEFSHEYWMRHALTLAKRARDGREVPVGAVLVLNNRVIGEGWNRAIGLHDPTAHAEIMALRQGGLVMQNYRLIDATLYVTFEPCVMCAGAMIHSRIGRVVFGVRNSKHGAAGSLVNVLNYPGMNHRVEITEGILADECAALLCDFYRMPRQVFNAQKKAQSSINSGGSSGGNSGSKTPGTSESATPESSGGSSGGSAKNTITKTLQLRIVRPYNSAEVEKIVTDEKNNREKIALEKNKDKVKEACSKHLKVASYCTTQVERNACLFCKARKLDDKFYQKLRGQFPDAVFWQEIGEIFRQLQKQAAEIYNQSLIELYYEIFIKGKGFANASSVEHYLSDVCYTRAAELFKNAAIASGLRGKVKSNFRLKELKNMKSGLPTTKSDNFPIPLVKQKGGQYTGFEISSHNDDLIIKIPFGRWQVRKEIDKYRPWEKFDFEQVRKSPKPICLLLSTQRRKRNKGWSKDEGTEAEIRKVMNGDYQTSYIEVKRGSRTGEKSAWMLNLSIDVPKIDKGVDPSVIGGIDVGVKSPLVCAINDAFSRYSISDNDLFHFNKKMFARRRILLKKNGRKRAGHGAKNKLKPITILTEKSKRFRKKLIERWACEIAGFFIKNRVGTVQMENLESMRRKEDSYFNIRLRGFWPYAEMQNKIEFKLKQYGIKIRKVAPNNTSKTCSKCGHLNNYFNFEYRKKNKFPHFKCEKCNFKENADYNAALNISNPKLKSTKEEP

SEQ ID NO: 1639 - protein, 726 aa, synthetic construct
SEVEFSHEYWMRHALTLAKRARDEREVPVGAVLVLNNRVIGVGWNRAVGLHDPTAHAEIMALRQGGLVMQNYRLIEATLYVTFEPCIMCAGAMIHSRIGRVVFGVRNSKRGAAGSLMNVLNYPGMNHRVEITEGILADECAALLCDYYRMPRQVFNARKKAQSSINSGGSSDGGSGSETPGASESVTPKSSGGSSAGSTKNTITKTLKLRIVRPYNSAEVEKIVADEKNNREKIALEKNKDKVKEACSKHLKVASYCTTQVERNACPFCKARKLDDKFYQKLRGQFPDAVFWQELGEILRQLQKQAAETYNQSLIELYYEIFIKGKGFANASSVEHYLSDVCYTRAAELFKNAAIASGLRGKVKSNFRLKELKNMKSGLPTTKSDNFPIPLVRQKGGQYTGFEISSHNDDFIIKIPFGRWQVRKEIDKYRPWEKFDFEQVRKSPKPISLLLSTQRRKRNKGWSKDEGTEAEIRKVMNGDYQTSYIEVKRGSKTGEKSAWMLNLSIDVPKIDKGVDPSIIGGIDVGVKSPLVCAINNALSRYSISDNDLFHFNKKMFARRRILLKKNGHKRAGHGAKNKLKPITIMTEKSKRFRKKLIERWACEIADFFIKNKVGTVQMENLESMKRREDSYFNIRLRGFWPYAEMQNKIEFKLKQYGIKIRKVAPNNTSKTCSKCGHLNNYFSFEYRKKNKFPHFKCEKCNFKEDADYNAALNISNPKLKSTKEEP

SEQ ID NO: 1640 - protein, 726 aa, synthetic construct
SEVEFSHEYWMRHALTLAKRARDGREVPVGAVLVLNNRVIGEGWNRAIGLHDPTAHAEIMALRQGGLVMQNYRLSGATLYVTFEPCVMCAGAMIHSRIGRVVFGVRNGKRGAAGSLMNVLNYPSMNHRVETTEGILADECAALLCDFYRMPRRVFNAQKKAQSSINSGGSSGGSGGSAPRGTSESATPESSGGSSGGSAKNTITKTLKLRIVRPYNSAEVEKIVADEKNNREKIALEKNKDKVREACSEHLKVAAYCTTQVERSACLFCKARKLDDKFYQKLRGQYPDAVFWQEIGEIFRQLQKQAAEIYNQSLIELYYEIFIKGKGFANASSVEHYLSDVCYTRAAELFKNAAIASGLRGKVKSNFRLKELKNMKSGLPTTKSDNFPIPLVKQKGGQYTGFEISSHNDDFIIKIPFGRWQVKKEIDRYRPWEKFDFEQVRKSPKPISLLLSTQRRKRNKGWSKDEGTEAEIRKVMNGDYQTSYIEVKRGSKIGEKSAWMLSLSIDVPKIDKGVDPSTIGGIDVGVKSPLVCAINNAFCRYSISDNDLFHFNKKMFARRRILLKKSRHKRAGHGAKNKLKPISILTEKSKRFRKKLIERWACEIADFFIKNKVGTVQMENLESMKRKEDSYFNIRLRGFWPYAEMQNKIEFKLKQYGIEIRKVAPNNTSKTCSKCGHLNNYFNFEYRKKNKFPHFKCEKCNFKENADYNAALNISNPKLKSTKEEP

SEQ ID NO: 1641 - protein, 726 aa, synthetic construct
SEVEFSHEYWMRHALTLAKRARDEREVPVGAVLVLNNRVIGEGWNRAIGLHDPTAHAEIMALRQGGLVMQNYRLIDATLYVTFEPCVMCAGAMIHSRIGRVVFGVRNNKRGAAGSLMNVLNYPGMNHRVEITEGILADECAALLCDFYRMPRQVLNAQKKARSSISPGGSSGGSSGSETPGASGSVTPKSSGGSSAGSTKDTITKTLKLRIVRPYNSAEVEEIVADEKNNRERIALEKNKDKVKEACSKHLKVAAYCTTQVERNACLFCKARKLDDKFYQKLRGQFPDAVFWQEIGEIFRQLQKQAAEIYNQSLIELYYEIFIKGKGFANASSAEHYLSDVCYTRAAELFKNAAIASGLRGKVKSNFRLKELKNMKSGLPTTKSDNFPIPLVKQKGGKYTGFEISSHNDDFIIKIPFGRWQVKKEIDKYRPWEKFDFEQVRKSPKPISLLLSTQRRKRNKGWSKDEGTEAEIRKVMNGDYQTSYIEVKRGSKIGEKSAWMLNLSIDVPKIDKGVDPSIIGGIDVGVKSPLVCAINNAFSRYSISDNDLFHFNKKMFARRRILLKKNRHKRAGHGAKNKLKPITILTEKSGRFRKKLIERWACEIADFFIKNKVGTVQMENLESMKRKEDSYFNIRLRGFWPYAEMQNKIEFKLKQYGIKIRKVAPNNTSKTCSKCGHLNNYFSFEYRKKNKFPHFKCEKCNFKENADYNAALNISNPKLMSTKEEP

SEQ ID NO: 1642 - protein, 726 aa, synthetic construct
SEDEFSHEYWMRHALTLAKRARDGREVPVGAVLVLNNRVIGEGWNRAIGLHDPTAHAEIMALRQGGLVMQNYRLIDATLYVTFEPCVMCAGAMVHSRIGRVVFGVRNSKRGAAGSLMNVLNYPGMNHCVEITEGILVDECAALLCDFYRMPRQVLNAQKKAQSSINPGGSSGGSSGSETPGTSESATPESSGGSSGSSAKNTITKTLKLRIVRPYNSAEVEKIVADEKNNREKIALEKNKDKVKEACSKHLKVATYCTTQVERNACLFCKARKLDDKFYQKLRGQFPDAVFWQEVGEIFRQLQKQAAEIYNQSLIELYYEIFIKGKGITNASRVEHYLSDVCYTRAAELFKNAAIASGLRGKVKSNFRLKELKNMKSGLPTTKSDNFPIPLVKQKGGQYTGFEISSHSDDFIIKIPFGRWQVRKEIDKYRPWEKFDFEQVRKSPKPISLLLSTQRRKRNKGWSKDEGTEAEIRKVMNGDYQTSYIEVKRGGKTGEKSAWMLNLSIDVPKIDKGVDPSIIGGIDVGVKSPLVCAINNAFSRYSISDNDLFRFNKRMFARRRILLKKNRHKRAGHGAKNKLKPISILTGKSERFRKKLIERWACEIADFFIKNKVGTVQMENLESMKRKEDSYFNIRLRGFWPYAEMQNKIEFKLKQYGIKVRKVAPNNTSKTCSKCGHLNNYFSFEYRKKNKFPHFKCEKCNFKENADYNAALNISNPKLKSTKEEP

SEQ ID NO: 1643 - protein, 726 aa, synthetic construct
SEVEFSHEYWMRHALTLAKRARDEREVPVGAILVLNNRVIGEGWNRAIGLHDPTAHAEIMALRQGGLVMQNYRLIDATLYVTFEPCVMCAGAMVHSRIGRVVFGVRNSKHGAAGSLVNVLNYPGMNHRVEITEGILADECAALLCDFYRMPRQVFNARKKAQSSINSGGSSGGSSGSETPGTSESATPESSGGSSGGSAKNTITKTLQLRIVRPYNSAEVERIVTDEKNNREKIALEKNKDKVKEACSKHLKMASYCTTQVERNACLFCKARKLDDKFYQKLRGQFPDAVFWQELGGIFRQLQKQAAEIYNQSLIELYYEIFIKGKGITNASRVEHYLSDVCYTRAAELFKNAAIASGLRSKVRSNFRLKELKNMKSGLPTTKSDNFPIPLVKQKGGQYTGFEISSHNSDFIIKIPFGRWQVKEEIDKYRPWEKFDFEQVRKSPKPISLLLSTQRRQKNKGWSEDEGTEAEIRRVMNGDYQTSYIEVKRGSKIGEKGTWTLNLSIDVPKIDKGVDPSIVGGIDVGVKSPLVCAINNSFSRYSICDNDLFRFNKKMFARRRILLKKNRHKRAGHGAKNKLKPITILTKKSERFRKKLIERWVCEVADFFIKNKVGTVQMENLESMKRKEDSYFNIRLRGFWPYAEMQNRIELKLKQYGIETRRVAPNNTSRTCSKCGHLNNYFSFEYRKKNKFPHFKCEKCNFREDADYNAALNISNPKLKSTKEEP

SEQ ID NO: 1644 - protein, 726 aa, synthetic construct
SEVEFSHEYWMRHALTLAKRARDEREVPVGAVLVLDNRVIGVGWNRAIGLHDPTAHAEIMALRQGGLVMQNYRLTDATLYVTFEPCVMCAGAMVHSRIGRVVFGVRNSKRGAAGSLMNVLNYPGMSHCVEITEGILADECAALLCDYYRMPRQVFNARKKAQSNINPGGPSGGSSGSETPDTSESATPESSGGNTGGSAKNTITKTLKLRIVRPYNSAEVEKIVADEKNNREKIALEKNKDKVKEACSEHLKVAAYCTTQVERNACLFCKARKLDDKFYQKLRGQFPDAVFWQELGEIFRQLQKQTAEIYNQSLIELYYEIFIKGKGFANASSVEHYLSDVCYTRAAELFKNAAIASGLRGKVKSNLRLKELKNMRSGLPTTKSDNFPIPLVKQKGGQYTGFEISSHNDDFIIKIPFGRWQVKKEIDKYRPWEKFDFEQVRKSPKPISLLLSTQRRKRNKGWSKDEGTEAEIRKVMNGDYQTSYIEVKRGSKIGEKSAWMLNLSIDVPKIDKGVDPSIIGGIDVGVKSPLVCAINNALSRYSISDNDLFHFNKKMFARRRILLRKNRHKRAGHGAKNKLKPITIMTEKSKRFRKKLIERWAREIADFFIKNKVGTVQMENLESMKRREDSYFNVRLRGFWPYAEMQNKIEFKLKQYGIEVRKVAPNNTSKTCSKCGHLNHYFNFEYRKKNKFPHFKCEKCNFKENADYNAALNISNPKLKSTKGEP

SEQ ID NO: 1645 - protein, 726 aa, synthetic construct
SEVEFSHEYWMRHALTLAKRARDEREVPVGAVLVLNNRVIGEGWNRAIGLHDPTAHAEIMALRQGGLVMQNYRLTDATLYVTFEPCVMCAGAMIHSRIGRVVFGVRNSKRGAAGSLMNVLNYPGMNHCVEITEGILVDECAALLCDFYRMPRQVLNAQKKAQSSISSGGSSGGCSGSEMPGASESVTPKSSGGSSAGSTKNTITKTLKLRIVRPYNSAEVEKIVADEKNSREKIALERNKDKVKEACSEHLKVAAYCTTQVERNACLFCKARKLDDRFYQKLRGQFPDAVFWQETGEIFRQLQRQAAEIYNQSLIELYYEIFIKGKGFANASSVEHYLSDVCYTRAAELFKNAAIASGLRGKVKSNFRLKELKNMKSGLPTTKSDNFPIPLVKQKGGQYTGFEISSHNSDFIIKIPFGRWQVKEEIDKYRPWEKFDFEQVRKSPKPISLLLSTQRRKKNKGWSKDEGTEAEIRKVMNGDYQTSYIEVKRGSKIGEKSAWMLNLSIDVPKIDKGVDPSIIGGIDVGVKSPLVCAINNSSSRYSICDNDLFRFNKKMFARRRILLKKNRHKRAGHGAKNKLKPITILTKKSERFRKKLIERWVCEVADFFIKNKVGTVQMENLESMKRKEDSYFNIRLRGFWPYAEMQNKIEFKLKQYGIKIRKVAPNNTSKTCSKCGHLNNYFSFEYRKKNKFPHFKCEKCNFKEDADYNAALNISNPKLKSTKEEP

SEQ ID NO: 1646 - protein, 726 aa, synthetic construct
SEVEFSHEYWMRHALTLAKRARDEREVPVGAILVLNNRVIGEGWNRAIGLHDPTAHAEIMALRQGGLVMQNYRLINATLYVTFEPCVMCAGAMIHSRIGRVVFGVRNSKRGAAGSLMNVLNYPGMNHRVEITEGILADECAALLCDYYRMPRQVFNARKKAQSSINSGGSSDGGSGSETQGTSESATPEGSGSSSGGSAKNTITKTLKLRIVRPYNSAEVEKIVADEKNNREKIALEKNKDKVKEACSKHLKVASYCTTQVERNACLFCKARKLDDKFYQKLRGQFPDAVFWQEIGEIFRQLQKQAAEIYNQSLIELYYEIFIKGKGFANASSVEHYLSDVCYTRAAELFKNAAIASGLRGKVKSNFRLKELKNMRSGLPTTKSDNFPIPLVRQKGGQYTGFEISNHDGDFIIKIPFGRWQVKKEINKHRPWEKFDFEQVRKSPKPISLLLSTQRRKRNKGWSKDEGTEAEIRKVMNGDYQTSYIEVKRGSKIGEKSAWMLNLSIDVPKIDKGVDPSIIGGIDVGVKSPLVCAINNALSRYSISDNDLFHFNKKMFARRRILLRKNRHKRAGHGAKNKLKPITMMTEKSKRFRKKLIERWACEIADFFIKNKVGTVQMENLESMKRKEDSYFNIRLRGFWPYAEMQDKIEFKLKQYGIVVRKVAPNNTSKTCSKCGHLNHYFNFEYRKKNKFPHFKCEKCNFKEDADYNAALNISNPKLKSTKGEP

SEQ ID NO: 1647 - protein, 726 aa, synthetic construct
SEVEFSHEYWMRHALTLAKRARDEREVPVGAILVLNNRVIGEGWNRAIGLHDPTAHAEIMALRQGGLVMQNYRLIDATLYVTFEPCVMCAGAMIHSRIGRVVFGVRNNKHGAAGSLVNVLNYPGMNHRVEITEGILADECAALLCDFYRMPRRVFNARRMAQSSIDPGGPSGGSGGSETPGTSESATPESSGGSSGGSAKNTITKTLKLRIVRPYNSTEVEKIVADEKDNREKIALEKNKDKVKEACSKHLKVASYCTTQVERNACLFCKARKLDDKFYQKLRGQFPDAVFWQELGEIFRQLQKQAAVIYNQSLIELYYEIFIKGKGIANASRVEHYLSDVCYTRAAELFKNAAVASGLRGKVKSNFRLKELKNMKSGLPTTKSDNFPIPLVKQKGGQYTGFEISSHNDDFIIKIPFGRWQVKKEIDKYRPWEKFDFEQVRKSPKPISLLLSTRRRKRNKGWSKDEGTEAEIRKVMNGDYQTSYIEVKRGSKTGEKSAWMLNLSIDVPKIDKGVDPSIIGGIDVGVKSPLVCAINNAFSRYSISDNDLFRFNKKMFARRRILLKKNRHKRAGHGAKNKLKPISILTEKSERFRKKLIERWACEIADFFIKNKVGIVQMENLESMKRREDSYFNIRLRGFWPYAEMQNKIEFKLKQYGIGIRKVAPNNTSKTCSRCGHLNNYFNFEHRKKNKFPRFKCEKCNFKENADYNAALNISNPKLKSTKEEP

SEQ ID NO: 1648 - protein, 726 aa, synthetic construct
TEVEFSHEYWMRHALTLAKRARDEREVPVGAVLVLNNRVIGEGWNRAIGLHDPTAHAEIMALRQGGLAMQNYRLVDATLYVTFEPCVLCAGAMVHSRIGRVVFGVRNNKRGAAGSLMNVLNYPGMNHRVEITEGILADECAALLCDFYRMPRQVFNAQKKARSNINSGGSSGGSSGSETPGTSESATPVSSSGSSGGSAKNTITKTLKLRIVRPYNSAEVEKIVADEKNNREKIALEKNKDRVKEACSKHLKVAAYCTTQVERNACPFCKARRLDDKFYQKLRGQFPDAVFWQEIGEIFRQLQKQAAEIYNQSLVELYYEIFIKGKGIANASSVEHYLSDVCYTRAAELFKNAAIASGLRNKIKSNFRLKELRNMKSGLPTTKSDNFPIPLVRQKGGQYTGFEISNHNGDFIIKIPFGRWQVKKEICKHRPWEKFDFEQVRKSPKPISLLLSTQRRKRNKGWGKDEGTEAEIRKVMNGDYQTSYIEVKRGSKIGEKSAWMLNLSIDVPKIDKGVDPSIIGGIDVGVKSPLVCAINNALSRYSISDNDLFHFNKKMFARRRILLRKNRHKRAGHGARNKLKPITVLTEKSERFRKKLIERWACEIANFFIKNKVGTVQMENLESMKRREDSYFNIRLRGFWPYAEMQSKIEFKLKQYGIKIRKVAPNNTSKTCSKCGHLNNYFNFEFRKKNKFPHFKCEKCNFKEDADYNAALNISNPKLKGTKEEP

SEQ ID NO: 1649 - protein, 726 aa, synthetic construct
SEVEFSHEYWMRHALTLAKRARDEREVPVGAILVLNNRVIGEGWNRAIGLHDPTAHAEIMALRQGGLVMQNYRLIDATLYVTFEPCVMCAGAMIHSRIGRVVFGVRNSKHGAAGSLVNVLNYPGMNHRVEITEGILADECAALLCDFYRMPRRVFNARMKAQSSISPGGPSGGSSGSETPSTSESATPESSGGSSGGSAKNTITKTLKLRIVRPYNSAEVEKIVADEKNNREKIALEKNKDKVKEACSEHLKVAAYCTTQVERNACLFCKARKLDDRFYQKLRGQFPDAVFWQETGEIFRQLQRQAAEIYNQSLIELYYEIFIRGKGFANASSVEHYLSDVCYTRAAELFKNAAIASGLRGKVKSNFRLKELKNMKSGLPTTKSDNFPIPLVKQKGGQYTGFEISSHNDDFIIKIPFGRWQVKKEIDKYRPWEKFDFEQVRKSPKPISLLLSTQRRKRNKGWSKDEGTEAEIRRVMNGDYQTSYIEVKRGSKIGEKSAWMLSLSIDVPKIDKGVDPSIIGGIDVGVKSPLVCAINNAFCRYSISDNDLFHFNKKMFARRRILLKKSRHKRAGHGAKNKLKPISILTEKSKRFRKKLIERWACEVADFFIKNKVGTVQMENLESMKRKEDSYFNIRLRGFWPYAEMQNKIEFKLKQYGIEIRKVAPNNTSKTCSKCGHLNSYFNFEYRKKNKFPHFKCEKCNFKENADYNAALNISNPKLKSTKEEP

SEQ ID NO: 1650 - protein, 726 aa, synthetic construct
SEVEFSHEYWMRHALTLAKRARDEREVPVGAVLVLNNRVIGEGWNRAIGLHDPTAHAEIMALRQGGLVMQNYRLTDATLYVTFEPCVMCAGAMIHSRIGRVVFGVRNSKHGAAGSLVNVLNYPGMNHRVEITEGILADECAALLCDFYRMPRQVFNAQGKAQSSTNSGGSSGGSSGSETPGTSESATPGSSGGSSGGSAKNTITKTLKLRIVRPYNSAEVEKIVADEKNSREKIALEKNKDKVREACSKHLRVAAYCTTQVERNACLFCKARKLDDKFYQKLRDQFPDAVFWQEIGEIFRQLQRQAAEIYNQSLIELYYEIFIKGKGFANASSVEHYLSDVCYTRAAELFKNAAIASGLRGKIKSNFRLKELKNMRSGLPTTKSDNFPIPLVKQKGGQYTGFEISSHNDDFIIKIPFGRWQAKEEINKYRPWEKFDFEQVRKSPKPISLLLSTQRRKRNKGWSKDEGTEAEIRKVMNGDYQTSYIEVKRGSKIGEKSAWMLNLSIDVPKIDKGVDPSIIGGIDVGVKSPLVCAINNAFSRYSISDNDLFHFNKKMFARRRILLKKTRHKRAGHGAKNKLKPISILTEKSERFRKKLIERWACEIADFFIKNKVGTVQMENLESMKRREDSYFSTRLRGFWPYAKMQNKIEFKLKQYGIEIRKVAPNNTSKTCSKCGHLNNYFNFEYRKKNKFPHFKCEKCNFKENADYNAALNISNPKLKSTKEEP

SEQ ID NO: 1651 - protein, 726 aa, synthetic construct
SEIEFSHEYWMRHALTLAKRARDEREVPVGAVLVLNNRVIGEGWNRAIGLHDPTAHAEIMALRQGGLVMQNYRLTDATLYVTFEPCVMCAGAMIHSRIGRVVFGVRNSKRGAAGSLMNVLNYPGMNHCVEITEGILVDECAALLCDFYRMPRQVLNAQKKAQSSISSGGSSGGSSCSETPGTSESATPESSGGGSSGSAKNTITKTLQLRIVRPYNSAEVEKIVADEKNNREKIALEKNKDKVKEACSEHLKVAAYCTTQVERSVCLFCKARKLDDKFYRKLRGQFPDAVFWQEIGEIFRQLQKQAAEIYNQSLIELYYEIFIKGKGIANASSVGHYLSDVCYTRAAELFKNAAIASGLRSKIKSNFRLKELRNMRGGLPTTKSDNFPIPLVKQKGGQYTGFEISSHNDDFIIKIPFGRWQVKKEIDKYRPWEKFDFEQVRKSPKPISLLLSTQRRKRNKGWSKDEGTEAEIRKVMNGDYQTSYIEVKRGSKIGEKSAWMLNLSIDVPKIDKGVDPSIIGGIDVGVKSPLVCAINNAFSRYSISDNDLFRFNKKMFARRRILLGKNRHKRAGHGVKNKLKPITILTEKSGRFRKKLIERWACEIADFFAKNKVGTVQMENLESMKRKEDSYFNIRLRGFWPYAEMQNKIEFKLKQYGIKVRKVAPNNTSKTCSRCGHLNNYFSFEYRKKNKFPHFKCEKCNFKENADYNAALNISNPKLKSTKEEP

SEQ ID NO: 1652 - protein, 726 aa, synthetic construct
SEVEFSHEYWMRHALTLAKRARDEREVPVGAILVLNNRVIGEGWNRAIGLHDPTAHAEIMALRQGGLVMQNYRLIDATLYVTFEPCVMCAGAMVHSRIGRVVFGVRNSKRGAAGSLMNVLDYPGMGHRVEITEGILADECAALLCDFYCMPRQVFNAQKRAQSSINSGGSSGGSSGSETPGTSESATPESSGGSSGGSAKNTITKTLKLRIVRPYNSAEVEKIVADEKNNREKIALEKNKDKVKEACSKHLKVASYCTTQVERNACLFCKARKLDDKFYQKLRGQFPDAVFWQELGEIFRQLQKQAAEIYNQSLIELYYEIFIKGKGFANASSVEHYLSDVCYTRAAELFKNAAIASGLRGKVKSNFRLKELKNMKSGLPTTKSDNFPIPLVKQKGGQYTGFEVSSHNDDFIIKIPFGRWQVKKEIDKYRPWEKFDFERVRKNPKPISLLLSTQRRKRNKGWSKDEGTEAEIRKVMNGDYQTSYIEVKRGSKIGEKSAWMLNLSIDVPKIDKGVDPSIIGGIDVGVKSPLVCAINNAFSRYSISDNDLYRFNKKMFARRRILLKKSKHKRAGHGAKNKLKPITILAEKSGRFRKKLIERWACEIADFFIKNKVGTVQMENLESMKRKEDSYFNIRLRGFWPYAEMQNKIEFKLKQYGIEIRKVAPNNTSKTCSKCGHLNNYFNFEYRKKNKFPHFKCEKCNFKENADYNAALNISNPKLKSTKEEP

SEQ ID NO: 1653 - protein, 726 aa, synthetic construct
SEDEFSHEYWMRHALTLAKRARDEREVPVGAILVLNNRVIGEGWNRAIGLHDPTAHAEIMALRQGGLVMQNYRLTDATLYVTFEPCVMCAGAMVHSRIGRVVFGVRNSKRGAAGSLMNVLNYPGVNHCVEITEGILVDECAALLCDFYRMPRQVLNAQKKAQSSISSGGSSGGCSGSEMPGASESVTPKSSGGSSAGSTKNAITKTLKLRIVRPYNSAEVEKIVADEKNSREKIALEKNKDKVKEACSRHLKVATYCTTQVERNACLFCKARKLDDKFYQKLRGQFPDAVFWQELGEIFRQLQKQAAEIYNQSLIELYYEIFIKGKGFANASSVEHYLSDVCYTRAAELFKNAAIASGLRGKVKSNFRLKELKNMKSGLPTTKSDNFPIPLVKQKGGQYTGFETSSHNDDFIIKIPFGRWQVKKEIDKYRPWEKFDFEQVRKSPKPISLLLSTQRRKRNKGWSKDEGTEAEIRKVMNGDYQTSYIEVKRGSKIGEKSAWMLNLSIDVPKIDKGVDPSIIGGIDVGVKSPLVCAINNAFSRYSISDNDLFRFNKKMFARRRILLKKNRHKRAGHGAKNKLKPISILTEKSKRFRKKLIERWACEIADFFIKNKVGTVQMENLESMKRKEDSYFNIRLRGFWPYAEMQNKIEFKLKQYGIEIRKVAPHNTSKTCSRCGHQNNYFNFEYRKKNKFPHFKCEKCNFKENADYNAALNICNPKLKGTKEEP

SEQ ID NO: 1654 - protein, 726 aa, synthetic construct
SEVEFSHEYWMRHALTLAKRARDEREVPVGAILVLNNRVIGEGWNRAIGLHDPTAHAEIMALRQGGLVMQNYRLIDATLYVTFEPCVMCAGAMIHSRIGRVVFGVRNNKHGAAGSLVNVLNYPGMNHRVEITEGILADECAALLCDFYRMPRQVFNARKKAQSSINSGGSSGGSSGSETPGASESVTPKSSGGNSGGSAKNTITKTLKLRIVRPYNSAEVEKIVADEKNNREKIALEKNKDKVKEACSEHLKVAAYCTTQVERSACLFCKARKLDDKFYQKLRDQFPDAVFWQEIGEIFRQLQRQAAEIYNQSLIELYYEIFIKGKGFANASSVEHYLSDVCYTRAAELFKNAAIASGLRGKVKSNFRLKELKNMKSGLPTTKSDNFPIPLVKQKGGQYTGFEISSHNDDFIIKIPFGRWQVKKEIDRYRPWEKFDFEQVRKSPKPISLLLSTQRRKRNKGWSKDVGTEAEIRKVMNGDYQTSYIEVKRGSKVGERSAWMLNLSIDVPKIDKGVDPSIIGGIDVGVKSPLVCAINNALSRYSISDNDLFHFNKKMFARRRILLRKNRHKRAGHGAKNKLKPITIMTEKSGRFRKKLIERWACEIANFFIKNKVGTVQMENLESMKRKEDSYFNIRLRGFWPYAEMQNKIEFKLKQYGIKIRKVAPNNTSKTCSKCGHLNNYFSFEYRKKNKFPHFKCEKCNFKEDADYNAALNISNPKLKSTKEEP

SEQ ID NO: 1655 - protein, 726 aa, synthetic construct
SEVEFSHEYWMRHALTLAKRARGEREVPVGAILVLNNRVIGEGWNRAIGLHDPTAHAEIMALRQGGLVMQNHRLVDATLYVTFEPCVMCAGAMIHSRIGRVVFGVRNSKHGAAGSLVNVLNYPGMNHRVEITEGILADECAALLCDFYRMPRQVFNARKKAQSSINPSGSSGGSSGSVTPGTSASATPESSGGSSAGSTKDTITKTLKLRIVRPYNSAEVEKIVADEKNNREKIALEKNKDKVKEACSKHLKVASYCTTQVERNACLFCKARKLDDKFYQKLRGQFPDAVFWQELGEIFRQLQKQAAEIYNQSLIELYYEIFIKGKGFANASSVEHYLSDVCYTRAAELFKNAAIASGLRGKVKSNFRLKELKNMKSGLPTTKSDNFPIPLVKQKGGQYTGFEICSHNDDFIIKIPFGRWQVKKEIDKYRPWEKFDFEQVRKSPKPISLLLSTQRRKRNKGWSKDEGTEAEIRKVMNGDYQTSYIEVKRGSKIGEKSAWMLSLSIDVPRIDRGVDPSIIGGIDVGVKSPLVCAINNALSRYSISDNDLYHFNKKMFARRRILLKKNRHKRTGHGARNKLKPITVLAEKSERFRKKLIERWACEIANFFIKNKVGTVQMENLESMKRKEDSYFNIRLRGFWPYAEMQNKIEFKLKQYGIEIRKVAPNNTSKTCSMCGHLNNYFNFEYRKRNKFPHFKCEKCNFKENADYNAALNISNPKLKSTKEEP

SEQ ID NO: 1656 - protein, 726 aa, synthetic construct
SEVEFSHEYWMRHALTLAKRARDEREVPVGAVLVLNNRVIGEGWNRAIGLHDPTAHAEIMALRQGGLVMQNYRLIDATLYVTFEPCIMCAGAMIHSRIGRVVFGVRNSKHGAAGSLVNVLNYPGMNHRVEITGGVLADECAALLCDFYRMPRQVFNAQKKAQSSINSGGSSGGSSGSETLSTSESATPESSGGSSGGSAKNTITKTLKLRIVRPYNSAEVEKIVADEKNNREKIALEKNKDKVKEACSEHLKVAAYCTTQVERSACLFCKARKLDDKFYQKLRGRFPDAVFWQELGEILRQLQKQAAEIYNQSLVELYYEIFIKGKGIANASSVEHYLSDVCYTRAAELFKNAAIASGLRNKIKSNFRLKELRNMKSGLPTTKSDNFPIPLVRQKGGQYTGFEISNHNGDFIIKIPFGRWQVKKEICKHRPWEKFDFEQVRKSPKPISLLLSTQRRKRNKGWGKDEGTEAEIRKVMNGDYHTSYIEVKRGSKIGEKSAWMLNLSIDVPKIDKGVDPSIIGGIDVGVKSPLVCAINNAFSRYSISDNDLFRFNKKMFARRRILLKKNRHKRAGHGAKNKLKPISILTGKSERFRKKLIERWACEIADFFIKNKVGTVQMENLESMKRKEDSYFNIRLRGFWPYAEMQNKIEFKLKQYGIEIRKVVPNNTSKTCSKCGHLNNYFNFEYRKKNKFPHFKCEKCNFKENADYNAALNISNPKLKSTKEEP

SEQ ID NO: 1657 - protein, 726 aa, synthetic construct
SEVEFSHEYWMRHALTLAKRARDEREVPVGAILVLNNRVIGEGWNRAIGLHDPTAHAEIMALRQGGLVMQNYRLIDATLYVTFEPCVMCAGAMIHSRIGRVVFGVRNSKHGAAGSLVNVLNYPGMNHRVEITEGILADECAALLCDFYRMPRQVFNARKKAQSSINPSGSSGGSSGSVTPGTSESATPESSGGSSGGSAKNTITKTLKLRIVRPYNSAEVEKVVADEKNNREKIALEKNKDKVKEACSKHLKVASYCTTQVERNACPFCKARKLDDKFYQKLRGQFPDAVFWQELGEILRQLQKQAAEIYNQSLIELYYEIFIKGRGFANASSVEHYLSDVCYTRAAELFKNAAIASGLRGKVKSNFRLKELKNMKSGLPTTKSDNFPIPLVKQKGGQYTGFEVSSHNGDFIIKIPFGRWQVKKEIDKYRPWEKFDFEQVRKSPKPISLLLSTQRRKRNKGWSKDEGTEAEIRKVMNGDYQTSYIEVKRGCKIGEKSAWMLNLSIDVPKIDKGVDPSIIGGIDVGVKSPLVCAINNAFSRYSISDNDLFHFNKKMFARRRILLKKNRHKRAGHGAKNKLKPISILTGKSERFRKKLIERWACEIADFFIKNKVGTVQMENLESMKRREDSYFNIRLRGFWPYAEMQNKIEFKLKQYGIEIRKVAPNNTSKTCSKCGHLNNYFNFEYRKKNKFPHFKCEKCNFKENADYNAALNISNPKLKSTKEEP

SEQ ID NO: 1658 - protein, 726 aa, synthetic construct
SEDEFSHEYWMRHALTLAKRARDEREVPVGAVLVLNNRVIGEGWNRAIGLHDPTAHAEIMALRQGGLVMQNYRLTDATLYVTFEPCVMCAGAMIHSRIGRVVFGVRNSKRGAAGSLMNVLNYPGMNHCVEITEGILMDECAALLCDFYRMPRQVLNAQKKAQSSISSGGSSGGSSGSETPGASESVTPKSSVGSSAGSTKNTITKTLKLRIVRPYNSAEVEKIVADEKNNREKIALEKNKDKVKEACSKHLKVAAYCTTQVERNACLFCKARKLDDKFYQKLRDQFPDAVFWQEISEIFRQLQKQAAEIYNQSLIELYYEIFIKGKGFANASSVEHYLSDVCYTRAAELFKNAAIASGLRGKVKSNFRLKELKNMKSGLPTTKSDNFPIPLVKQKGGQYTGFEISSHNDDFIIKIPFGRWQVKKEIDKYRPWEKFDFEQVRKSPKPISLLLSTQRRKRNKGWSKDEGTEAEIRKVMNGDYQTSYIEVKRGSKIGEKSAWMLNLSIDVPKIDKGVDPGIIGGIDVGVKSPLVCAINNAFSRYSISDNDLFHFNKKMFARRRILLQKNRHRRAGHGTKNKLKPITVLTEKSEGFRKKLIERWACEIADFFIKNKVGTVQMENLESMKRKEDSYFNIRLRGFWPYAEMQSKIEFKLRQYGIEIRKVAPNNTSKTCSKCGHLNNYFDFEYRKKNKFPHFKCEKCNFKENADYNAALNISNPKLKSTKEEP

SEQ ID NO: 1659 - protein, 726 aa, synthetic construct
SEVEFSHEYWMRHALTLAKRARDEREVPVGAVLVLNNRVIGEGWNRTTGLHDPTAHAEIMALRQGGLVMRNYRLTDATLYVTFEPCVMCAGAMIHSRIGRVVFGVRNSKRGAAGSLMNVLNYPGMNHCVEITEGILVDECAALLCDFYRMPRQVLNAQKKAQSSINPGGSSGGSSGSETPGTSESATPESSGGSSGSSAKNTITKTLQLRIVRPYNSAEVEKIVADEKNNREKIALEKNKDKVKEACSKHLKVASYCTTQVERNACPFCKARKLDDKFYQKLRSQFPDAVFWQELGEILRQLQKQAAEIYNQSLIELYYEIFIKGRGFANASSVEHYLSDVCYTRAAELFKNAAIASGLRGKVKSNFRLKELRNMRSGLPTTKSDNFPIPLVKQKGGQYTGFEISSHNDDFIIKIPFGRWQVKKEIDKYRPWEKFDFEQVRKSPKPFSLLLSTQRRKRNKGWSKDEGTEAEIRKVMNGDYQTSYIEVKRGSKVGEKSAWMLNLSIDVPKIDKGVDPSIIGGIDVGVKSPLVCAINNAFSRYSISDNDLFRFNKKMFARRRILLKKNRHKRAGHGAKNKLKPISILTGKSERFRKKLIERWACEIADFFIKNKVGTVQMENLESMKGKEDSYFNIRLRGFWPYAEMQNKIEFKLKQYGIKIRKVAPNNTSKTCSMCGHLNNYFSFEYRKKNKFPHFKCEKCNFKENADYNAALNISNPKLMSAKEGP

SEQ ID NO: 1660 - protein, 726 aa, synthetic construct
SEVEFSHEYWMRHALTLAKRARDEREVPVGAVLVLNNRVIGEGWNRAIGLHDPTAHAEIMALRQGGLVMQNYRLVDATLYVTFEPCVLCAGAMVHSRIGRVVFGVRNSKRGAAGSLMNVLNYPGMSHRVEITEGILADECAALLCDFYRMPRQVFNARKKARSNINSSGSSGGSSGSETPGTSESATPESSGGSSGGSAKNTITKTLKLRIVRPYNSAEVEKIVADEKNNREKIALEKNKDKVKEACSEHLKVAAYCTTQVERNACLFCRARKLDDKFYQKLRGQFPDAVFWQEIGEIFRQLQKQAAEIYNQSLIELYYEIFIKGKGFANASSVEHYLSDVCYTRAAELFKNAAIASGLRGKVKSNFRLKELKNMKSGLPTTKSDNFPIPLVKQKGGQYTGFEISSHNDDFIIKIPFGRWQVKKEIDKYRPWEKFDFEQVRRSPKPISLLLSTQRRKKNKGWSKDEGTEAEIRRVMNGDYQTSYIEVKRGSKIGEKSAWMLNLSIDVPKIDKGVDPSIIGGIDVGVKSPLVCAINNAFSRYSISDNDLFHFNKKMFARRRILLKKNRRRRAGHGAKNKLKPITILTEKSVRFRKKLIERWACEIADFFIKNKVGTVQMENLEGMKRKEDSYFNIRLRGFWPYAEMQNKIEFKLKQYGIEIRKVAPNNTSKTCSRCGHLNNYFNFEYRRKNKFPHFKCEKCNFKENADYNAALNISNPKLKSTKEEP

SEQ ID NO: 1661 - protein, 726 aa, synthetic construct
SEVEFSHEYWMRRALTLAKRARDEREVPVGAVLVLNNRVIGVGWNRAAGLHDPTAHAEIMALRQGGLVMQNYRLVEATLYVTFEPCIMCAGAMIHSRIGRVVFGVRNSKRGAAGSLMNVLNYPGMNHRVEITEGILADECAALLCDYYRMPRQVFNARKKAQSSINSGGSSDGGSGSETPGTSESATPESSGGSSGGSAKNTIIKTLKLRIVRPYNSAEVEKIVADEKNDREKIALEKNKDKVKEACSEHLKVAAYCTTQVERSACLFCKARKLDDKFYQKLRGQFPDAVFWQEIGEIFRQLQKQAAEIYNQSLIELYYEIFIKGKGFANASSVEHYLSDVCYTRAAELFKNAAIASGLRGKVKSNFRLKELKNMKSGLPTTKSDNFPIPLVKQKGGQYAGFEISSHNDDFIIKIPFGRWQVKKEIDKYRPWEKFDFEQVRKSPKPISLLLSTRRRKRNKGWSKDEGTEAEIRKVMNGDYQTSYIEVRRGSKIGEKSAWMLNLSIDVPKIDKGVDPSIIGGIDVGVKSPLVCAINNAFSRYSISDNELFHFNKKMFARRRILLKKNRHKRAGHGAKNKLKPITILTEKSGRFRKKLIERWACEIADFFIKNKVGTVQMENLESMKRKEDSYFNIRLRGFWPYAEMQNKIEFKLKQYGIEIRKVAPNNTSKTCSKCGHLNHYFNFEYRKKNKFPHFKCEKCNFKENADYNAALNISNPKLKSTKEEP

SEQ ID NO: 1662 - protein, 726 aa, synthetic construct
SEVEFSHEYWMRHALTLAKRARDEREVPVGAVLVLNNRVIGVGWNRAIGLHDPTAHAEIMALRQGGLVMQNYRLIDATLYVTFEPCVMCAGAMVHSRIGRVVFGVRNSKRGAAGSLMNVLDYPGMGHRVEITEGILADECAALLCDFYCMPRQVFNAQKRAQSSINSGGSSGGSSGSDTPGTSESATPESSGGGSSGSAKNTITKTLQLRIVRPYNSAEVEKIVADEKNNREKIALEKNKDKVKEACSKHLKVASYCTTQVERNACLFCKARKLDDKFYQKLRGQFPDAVFWQELGEIFRQLQKQAAEIYNQSLIELYYEIFIKGKGLANASSVEHYLSDVCYTRAAELFKNAAIASGLRGKVKSNFRLKELKSMKSGLPSTKSDNFPIPLVKQRGGQYTGFEISSHNDDFIIKIPFGRWQAKKEIDKYRPWEKFDFEQVRKSPKPISLLLSTQRRKRNRGWSKDEGTEAEIRKVMNGDYQTSYIEVKRGSKIGEKSAWMLNLSIDVPRIDKGVDPSIIGGIDVGVKSPLVCAINNAFSRYSISDNDLFRFNKKMFARRRILLGKNRHKRAGHGVKNKLKPITILTEKSGRFRKKLIERWACEIADFFVKNKVGTVQMENLESMKRKEDSYFNIRLRGFWPYAEMQNKIEFKLKQYGIKVRKVAPNSTSKTCSKCGHLNNYFSFEYRKKNKFPHFKCEECNFKENADYNAALNISNPKLKSTKEEL

SEQ ID NO: 1663 - protein, 726 aa, synthetic construct
SEVEFSHEYWMRHALTLAKRARDEREVPVGAVLVLNNRVIGEGWNRAIGLHDPTAHAEIMALRQGGLVMQNYRLTDATLYVTFEPCVMCAGAMIHSRIGRVVFGVRNSKRGAAGSLMNVLNYPGMNHCVGITEGILVDECAALLCDFYHMPPQVLNARKKAQSSISSGGSSGGSSGSETPGTSESATPESSGGSSGGSAKNTITKTLKLRIVRPYNSAEVEKIVADEKNSREKIALEKNKDKVKEACSKHLKVAAYCTTQVERNACLFCKARRLDDKFYQKLKGQFPDAVFWQEIGEVFRQLQKQAAEIYNQSLIELYYEIFIKGKGFANASSVEHYLSDVCYTRAAELFKNAAIASGLRGKVKSNFRLKELKNMKSGLPTTKSDNFPIPLVKQKGGQYTGFEISSHNSDFIIKIPFGRWQEKEEIDKYRPWEKFDFEQVRKSPKPISLLLSTQRRKRNKGWSKDEGTEAEIRKVMNGDYQTSYIEVKRGSKIGEKSAWMLNLSIDVPKIDKGVDPSIIGGIDVGVKSPLVCAINNAFSRYSISDNDLFHFNKKVFARRRILLKKNRHRRAGHGAKNKLKPITILTEKSKRFRKKLIERWACEIADFFIKNKVGTVQMENLESMKRKEDSYFNIRLRGFWPYAEMQNKIEFKLKQYGIKIRKVAPNNTSRTCSECGHLNNYFSFEYRKKNKFPHFKCEKCNFKENADYNAALNISNPKLKSTKEEP

SEQ ID NO: 1664 - protein, 726 aa, synthetic construct
SEIEFSHEYWMRHALTLAKRARDEREVPVGAVLVLNNRVIGEGWNRAIGLHDPTAHAEIMALRQGGLVTQNYRLIDATLYVTFEPCAMCAGAMVHSRIGRVVFGVRNSKRGAAGSLMNVLNYPGMDHRVEITGGILADECAALLCDFYRMPRRVFNAQKKAHSSINPGGSSGGSSGSVTPGTSESATPESSGGSSGGSAKNTITKTLKLRIVRPYNSAEVEKIVADEKNNREKIALEKNKDKVKEACSKHLKVAAYCTTQVERNACLFCKARKLDDKFYRKLKGQFPDAVFWQEIGEIFRQLQKQAAEIYNQSLIELYYEIFIKGKGFANASSVEHYLSDVCYTRAAELFKNAAIASGLRNKIKSNFRLKELRNMKSGLPTTKSDNFPIPLVRQKGGQYTGFEISNHDGDFIIKIPFGRWQVKKEINKHRPWEKFDFEQVRKSPKPISLLLSTQRRKRNKGWSKDEGTEAEIRKVMNGDYQTSYIEVKRGSKIGEKSAWMLNLSIDVPKIDKGVDPSIIGGIDVGVKSPLVCAINNALSRYSISDNDLFHFNKKMFARRRILLRKNRHKRAGHGAKNKLKPITIMTEKSKRFRKKLIERWACEIADFFIKNKVGTVQMENLESMKRREDSYFNIRLRGFWPCAEMQNKIEFKLKQYGIVVRKVAPNNTSKTCSKCGHLNNYFNYEYRKMNKFPHFKCEKCNFKEDADYNAALNISNPKLKSTKEEP

SEQ ID NO: 1665 - protein, 726 aa, synthetic construct
SEVEFSHEYWMRHALTLAKRARDEREVPVGAILVLNNRVIGEGWNRAIGLNDPTAHAEIMALRQGGLVMQNYRLIDATLYVTFEPCVMCAGAMIHSRIGRVVFGVRNNKHGAAGSLVNVLNYPGMNHRVEITEGILADECAALLCDFYRMPRQVFNARKKAQSSINPGGSSGGSGGSETPGTSESATPESSGGSSGSSAKNTITKTLKLRIVRPYNSAEVEKIVADEKNNREKIALEKNKDKVKEACSKHLKVAAYCTTQVERNACLFCKARRLDDKFYQKLRGQFPDAVFWQEIGEILRQLQKQAAEIYNQSLIELYYEIFIKGRGFANASSVEHYLSDVCYTRAAELFKNAAIASGLRGKVKSNFRLKELKNMKSGLPTTKSDNFPIPLVKQKGGQYTGFEISSHNDDFIIKIPFGRWQVKKEIDKYRPWEKFDFEQVRKSPKPISLLLSTQRRKRNKGWSKDEGTEAEIRKVMNGDYQTSYIEVKRGSRTGEKSAWMLNLSIDVPKIDKGVDPSIIGGIDVGVKSPLVCAINNAFSRYSISDNDLFRFNKKMFARRRILLKKNRHKRAGHGAKNKLKPISILTGKSERFRKKLIERWACEIADFFIKNKVGTVQMENLESMKRKEDSYFNIRLRGFWPYAEMQNKIEFKLKQYGIEIRKVAPNNTSKTCSKCGHLNNYFNFEYRKKNKFPHFKCEKCNFKENADYNAALNISNPKLKSTKEEP

SEQ ID NO: 1666 - protein, 726 aa, synthetic construct
SEVEFSHEYWMRHALTLAKRARDEREVPVGAVLVLNNRVIGEGWNRAIGLHDPTAHAEIMALRQGGLVMQNYRLSDATLYVTFEPCVMCAGAMIHSRICRVVFGVRNSKRGAAGSLMNVLNYPGMNHCVEITEGILVDECAALLCDFYRMPRQVLSAQKKAQSSISSGGSSGGSSGSETPGTSESATPENSGGSSGSSAKNTITKTLKLRIVRPYNSAEVEKIVADEKNNREKIALEKNKDKVKEACSKHLKVAAYCTTQVERNACLFCKARKLDDKFYQELRGQCPDAVFWQEIGEVFRQLQKQAAEIYNQSLIELYYEIFIKGKGFANASSVEHYLSDVCYTRAAELFKNAAIASGLRGKVKSNFRLKELKNMKSGLPTTKSDNFPIPLVKQKGGQYTGFEISSHNDDFIIKIPFGRWQVKKEIDKYRPWEKFDFEQVRKSPKPISLLLSTQRRKRNKGWSKDEGTEAEIRKVMNGDYQTSYIEVKRGSKIGEKSAWTLSLSIDVPKIDKGVDPSIIGGIDVGVKSPLVCAINNAFCRYSISDNDLFHFNKKMFARRRILLKKSRHKRAGHGAKNKLKPISILTEKSKRFRKKLIERWACEIADFFIKNKVGTVQMENLESMKRKEDSYFNIRLRGFWPYAEMQNKIEFKLKQYGIEIRKVAPNNTSKTCSKCGHLNNYFNFEYRKKNKFPHFKCEKCSFKENADYNAALNISNPKLKSTREEP

SEQ ID NO: 1667 - protein, 726 aa, synthetic construct
SEVEFSHEYWMRHALTLAKRARDEREVPVGAVLVLNNRVIGEGWNRAIGLHDPTAHAEIMALRQGGLVMQNYRLIDATLYVTFEPCVMCAGAMIHSRIGRVVFGIRNNKHGAAGSLVNVLDYPGMNHRVEITEGILADECAALLCDFYRMPRQVFNAQKKARPNINSGGSSGGRSGSETPGTSESATPESSGGSSGGSAKNTITKTLKLRIVRPYNSAEVEKIVADEKNNREKIALEKNKDKVKEACSKHLKVAAYCTTLVERNACLFCKARKLDDEFYQKLRGQFPDAVFWQEISEIFRQLQKQAAEIYNQSLVELYYEIFIKGKGIANASSVEHYLSDVCYTRAAELFKNAAIASGLRNKIKSNFRLKELRNMKSGLPTTKSDNFPIPLVRQKGGQYTGFEISNHNGDFIIKIPFGRWQVKKEISKHRPWEKFDFEQVRKSPKPISLLLSTQRRKRNKGWGKDEGTEAEIRKVMNGDYQTSYIEVKRGSKIGEKSAWMLNLSIDVPKIDKGVDPSIIGGIDVGVKSPLVCAINNALSRYSISDNDLFRFNKKMFARRRILLKKNRHKRAGHGAKNKLKPLSILTEKSERFRKKLIERWACEIADFFIKNKVGTVQMENLESMKRKEDSYFNIRLRGFWPYAEMQDKIEFKLKQYGIAIRKVAPNNTSKTCSKCGHLNNYFNFEYRKKNRFPHFKCEKCNFKENADYNAALNISNPKLKSTKEEP

SEQ ID NO: 1668 - protein, 726 aa, synthetic construct
SEVEFSHEHWMRHALTLAKRARDEREVPVGAVLVLNNRVIGEGWNRTTGLHDPTAHAEIMALRQGGLVMQNYRLIDATLYVTFEPCVMCAGAMIHSRIGRVVFGVRNNKHGAAGSLVNVLNYPGMNHRVEITEGILADECAALLCDFYRMPRQVFNARKKAQSSINPGGPSGGSSCSETPGASESVTPKSSGGSSTGSTKNTITKTLKLRIVRPYNSAEVEKIVADEKNSREKIALEKNKDKVKEACSKHLKVASYCTTQVERNACLFCKARKLDDKFYQKLRGQSPDAVFWQELGEIFRQLQKQAAEIYNQSLIELYYEIFIKGKGFANASSVEHYLSDVCYTRAAELFKNAAIASGLRNKIKSNFRLKELRNMKSGLPTTKSDNFPIPLVRQKGGRYTGFEISNHNGDFIIKIPFGRWQVKKEINKHRPWEKFDFEQVRKSPKPISLLLSTQRRKRNKGWSKDEGTEAEIRKVMNGDYRTSYIEVKRGNKIGEKSAWMLNLSIDVPKIDKGVDPSIIGGIDVGVKSPLVCAINNAPSRYSISDNDLFHFNKKVFARRRILLKKNRHKRAGHGARNKLKPITVLTEKSERFRKKLIERWACEIAYFFIKNKVGTVQMEDLESMKRKEDSYFNIRLRGFWPYAEMQNKIEFKLKQYGIEVRKVAPNNTSKTCSKCGHLNSYFNFEYRKKNKFPHFKCEKCNFKEDADYNAALNISNPKLKSTKEEP

SEQ ID NO: 1669 - protein, 726 aa, synthetic construct
SEVEFSHEYWMRHALTLAKRARDEREVPVGAVLVLNNRVIGEGWNRAIGLHDPTAHAEIMALRQGGLVMQNYRLSDATLYVTFEPCVMCAGAMIHSRIDRVVFGVRNSKRGAAGSLMNVLNYPGMNHCVEITEGILVDECAALLCDFYRMPRQVLSAQKKAQSSISSGGSSGGSSGSETPGASGSVTPKSSVGSSAGSTKNTITKTLKLRIVRPYNSAEVEKIVADEKNNREKIALEKNKDKVKEACSKHLKVASYCTTQVERNACPFCKARKLDDKFYQKLRGQFPDAVFWQELGEILRQLQKQAAEIYNQSLIELYYEIFIKGRGFANASSVEHYLSDVCYTRAAELFKNAAIASGLRGKVKGNFRLKELKNMKSGLPTTKSDNFPIPLVKQKGGQYTGFEISSHNDDFIIKIPFGRWQAKKEIDKYRPWEKFDFEQVRKSPKPISLLLSTQRRKRNKGWSRDEGTEAEIRKVMSGDYQTSYIEVKRGSKVGEKSAWMLNLSIDVPKIDRGVDPSIIGGIDVGVKSPLVCAINSAFSRYSIGDNDLFHFNKKMFARRRLLLKKNRHKRAGHGARNKLKPITTLTEKSEKFRKKLIERWACEIADFFTKNKVGTVQMENLESMKRKEDSYFNIRLRGFWPYAEMQNKIEFKLEQYGIVVRKVAPNNTSKTCSKCGHLNNYFNFEYRKKNKFPHFKCEKCNFKENADYNAALNISNPKLKSTKGEP

SEQ ID NO: 1670 - protein, 726 aa, synthetic construct
SEVEFSHEYWMRHALTLAKRARDEREVPVGAVLVLNNRVIGEGWNRAIGLHDPTAHAEIMALRQGGLVMQNYRLTDATLYVTFEPCVMCAGAMIHSRIGRVVFGVRNSKRGAAGSLMNVLNYPGMNHCVEITEGILVDECAALLCDFYRMPRQVLNTQKKAQSSISSGGSSGGCSGSEMPGASESVTPKSSGGSSGGSAKNTITKTLKLRIVRPYNSAEVEKIVADEKNNREKTALEKNKGKVKEACSEHLKVAAYCTTQVERNACPFCKARKLDDKFYQKLRGQFPDAVFWQEIGEIFRQLQKQAAEVYNQSLIELYYEIFIKGKGFANASSAEHYLSDVCYTRAAELFKNAAIASGLRGKVKSNFRLKELKNMKSGLPTTKSDNFPIPLVRQKGGQYTGFEISSHNDDFIIKIPFGRWQVKKEIDKYRPWEKFDFEQVRKSPKPISLLLSTQRRKRNKGWSKDEGTEAEIRKVMNGDYQTSYIEVKRGSKIGEKSAWMLNLSIDVPKIDKGVDPSIIGGIDVGVKSPLVCAINNAFSRFSISDNDLFHFNKKMFARRRILLKKNRHRRAGHGVKNKLKPITILAEKSKRFRKKLIERWACEIADFFVKNKVGTVQMENLESMKRKEDSYFNIRLRGFWPYAEMQNKIEFKLKQYGIEIRKVAPNNTSRTCSKCGHLNNYFNFEYRKKNKFPHFKCEKCNFKENADYNAALNISNPKLKGTKEEP

SEQ ID NO: 1671 - protein, 726 aa, synthetic construct
SEVEFSHEYWMRHALTLAKRARDEREVPVGAILVLNNRVIGEGWNRAIGLHDPTAHAEIMALRQGGLVMQNYRLTDATLYVTFEPCVMCAGAMIHSRIGRVVFGVRNSKRGAAGSLLNVLNYPGMNHCVEITEGILVDECAELLCDFYRMPRQVLNAQKKAQSSISSGGSSGGSSGSETPGASESATPKSSGGSSASSTKNTITKTLKLRIVRPYNSAEVEKIVADEKNNRERIALEKNKDKVKEACSKHLKVAAYCTTQVERNACLFCKARKLDDKFYQKLRGQFPDAVFWQEIGEIFRQLQKQAAEIYNQSLIELYYEIFIKGKGFANASSVEHYLSDVCYTRAAELFKNAAIASGLRGKVKSNFRLKELKNMRSGLPTAKSDNFPIPLVKQKGGQYTGFEISSHNDDFIIKIPFGRWQVKKEIDKYRPWEKFDFEQVRKSPKPISLLLSTRRRKRNKGWSKDEGTEAEIRKVMNGDYQTSYIEVKRGSKIGEKSAWMLNLSIDVPKVDKGVDPSIIGGIDVGVKSPLVCAINNAFSRYSISDNELFHFNKKMFARRRILLKKNGHKRAGHGVKNKLRPITILAEKSERFRKKLIEKWACEIADFFIKNKVGTVQMENLESMKRKEDSYFNIRLRGFWPYAEMQNKIEFKLKQYGIEVRKVAPNNTSKTCSECGHLNNYFNFEYRKKNKFPHFKCEKCNFKEDADYNAALNISNPKLKSTKEEP

SEQ ID NO: 1672 - protein, 726 aa, synthetic construct; identical to SEQ ID NO: 684

SEQ ID NO: 1673 - protein, 726 aa, synthetic construct
SEVEFSHEYWMRRALTLAKRARDEREVPVGAVLVLNNRVIGVGWNRAVGLHDPTAHAEIMALRQGGLVMQNYRLIEATLYVTFEPCIMCAGAMIHSRIGRVVFGVRNSKRGAAGSLMNVLNYPGMNHRVEITEGILADECAALLCDYYRMPRQVFNARKKAQPSANSGGSSDGGSGSETPGTSESATPESSGGSSGGSAKNTITKTLKLRIVRPYNSAEVEKIVADEKSNREKIALEKNKDKVKEACSEHLKVAAYCTTQVERSACLFCKARKLDDKFYQKLRGQFPDAVFWQEIGEIFGQLQRQAAEIYNQSLIELYYEIFIKGKGFANASSVEHYLSDVCYTRAAELFKNAAIASGLRGKVKSNFRLKELKNMKSGLPTTKSDNFPIPLVKQKGGQYTGFEISSHNDDFIIKIPFGRWQAKKEIDKYRPWEKFDFEQVRKSPKPISLLLSTRRRKRNKGWSKDEGTEAEIRRVMNGDYQTSYIEVKRGSKIGEKSAWVLNLSIDVPKIDKGVDPSIIGGIDVGVKSPLVCAINNAFSRYSISDNDLFRFNKKMFARRRILLKKNRHKRAGHGAKNKLKPISILTGKSERFRKKLIERWACEIADFFTKNKVGTVQMENLESMKRREDSYFNIRLRGFWPYAEMQNKIEFKLKQYGIEIRKVAPNNTSKTCSKCGHLNNYFNFEYRKKNKFPYFKCEKCNFKENADYNAALNISNPKLKSTREEP

SEQ ID NO: 1674 - protein, 726 aa, synthetic construct
SEVEFSHEYWMRHALTLAKRARDEREVPVGAILVLNNRVIGVGWNRAIGLHDPTAHAEIMALRQGGLVTQNYRLTDATLYVTFEPCVMCAGAMIHSRIGRVVFGVRNSKRGAAGSLMNVLNYPGMNHCVEITEGILVDECAALLCDFYRMPRQVLNAQKKAQSSISSGGSSGGSSGSETPGASGSVTPKSSGGSSACSTKDTITKTLKLRIVRPYNSAEVEKIVADEKNSREKIALEKNKDKVKEACSEHLKVAAYCTTQVERNACLFCKARKLDDRFYQKLRGQFPDAVFWQEIGEIFRQLQKQAAEIYNQSLIELYYEIFIKGKGFANASSVEHYLSDVCYTRAAELFKNAAIASGLRGKVKSNFRLKELKNMKSGLPTTKSDNFPIPLVKQKGGQYTGFEISSHNDDFIIKIPFGRWQVKKEIDKYRPWEKFDFEQVRKSPKPISLLLSTQRRKRNKGWSKDEGTEAEIRKVMNGDYQTSYIEVKRGSKIGEKSAWMLNLSIDVPKIDKGVDPRIIGGIDVGVKSPLVCAINNAFSRYSISDNDLFHFNKKVFARRRILLKKNRHRRAGHGARNKLKPITVLTEKSERFRKKLIERWACEIANFFIKNKVGTVQMENLESMRRKEDSYFNIRLRGFWPYAEMQSKIEFKLKQYGIEIRKVAPNNTSKTCSKCGHLNNYFNFEYRKKNKFPHFKCEKCNFKENADYNAALNISNPKLKSTREEP

SEQ ID NO: 1675 - protein, 726 aa, synthetic construct
SEVEFSHEYWMRHALTLAKRARDEREVPVGAILVLNNRVIGVGWNRAIGLHDPTAHAEIMALRQGGLVMQNYRLIDATLYVTFEPCVMCAGAMIHSRIGRVVFGVRNSKHGAAGSLVNVLNHPGMNHRVEITEGILADECAALLCDFYRMPRQVFNARKKVQSSINSGGSSGGSSGSETPGTSESATPKSSGGSSGGSAKNTITKALKLRIVRPYNSAEVEKIVADEKNNRERIALEKNKDKVKEACSKHLKVAAYCTTQVERNACLFCKARKLDDKFYQKLRGQFPDAVFWQEIGEIFRQLQRQAAEIYNQSLIELYYEIFIKGRGSANASSVEHYLSDVCYTRAAELFKNAAIASGLRGKVKGNFRLKELKNMKSGLPTTKSDNFPIPLVKQKGGQYTGFEISSHNDDFIIKIPFGRWQVKKEIDKYRPWEKFDFEQVRKSPKPISLLLSTQRRKRNKGWSKDEGTEAEIRKVMSGDYQTSYIEVKRGSKTGEKSAWMLNLSIDVPKIDKGVDPSIIGGIDVGVKSPLVCAINNAFSRYSISDNDLFRFNKKMFARRRILLKKNRHKRAGHGAKNKLKPITILTEKSVRFRKKLIERWACEIADFFIKNKVGTVQMENLESMKRKEDSYFNIRLRGFWPYAEMQNKIEFKLKQYGIKIRKVAPNNTSKTCSKCGHLSNNFSFEYRKKNKFPHFKCEKCNFKEDADYNAALNISNPKLKSTKEEP

SEQ ID NO: 1676 - protein, 726 aa, synthetic construct
SEVEFSHEYWMRHALTLAKRARDEREVPVGAILVLNNRVIGEGWNRAIGLHDPTAHAEIMALRQGGLVMQNYRLTDATLYVTFEPCVMCAGAMIHSRIGRVVFGVRNSKRGAAGSLMNVLNYPGMNHCVEITEGILVDECAALLCDFYRMPRQVLNAQKKAQSSISSGGSSGGSSGSETPGASESATPESSGGSSGSSAKNTITKTLKLRIVRPYNSAEVEKIVADEKNNREKIALEKNKDKVKEACSKHLKVAAYCTTQVERNACLFCKARRLDDKFYQKLRGQFPDAVFWQELGEILRQLQKQAAEIYNQSLIELYYEIFIKGRGFANASSVEHYLSDVCYTRAAELFKNAAIASGLRGKVKSNFRLKELKNMKSGLPTTKSDNFPIPLVKQKGGQYTGFEISSHNDDFIIKIPFGRWQVKKEIDKYRPWEKFDFEQVRKSPKPISLLLSTQRRKRNKGWSKDEGTEAEIRKVMSGDYQTSYIEVKRGSKTGEKSAWMLNLSIDVPKIDKGVDPSIIGGIDVGVKSPLVCAISNAFSRYSISDNDLFRFNKKMFARRRILLKKNRHKRAGHGAKNKLKPISILTGKSERFRKKLIERWACEIADFFIKNKVGTVQMENLESMKKKEDSYFNIRLRGFWPYAEMQNKIEFKLKQYGIEIRKVAPNNTSKTCSKCGHLNNYFNFEYRKRNKFPHFKCEKCNYKENADYNAALNISNPKLKSTKEEP

SEQ ID NO: 1677 - protein, 726 aa, synthetic construct
SEVEFSHEYWMRHALTLAKRARDEREVPVGAILVLNNRVIGEGWNRAIGLHDPTAHAEIMALRQGGLVMQNFRLIDATLYVTFEPCVMCAGAMIHSRIGRVVFGVRNNKHGAAGSLVNVLDHPGMNHRVEITEGILADECAALLCDFYRMPRQVFNARKKAQSSISPGGSSGGSSGSETPGTSESATPESSGGSSGGSAKNTITKTLKLRIVRPYNSAEVEKIVADEKNNREKIALEKNKDKVKEACSKHLKVAAYCTTQVERNACLFCKARKLDDKFYQKLRGQFPDAVFWQEIGEVFRQLQKQAAEIYNQSLIELYYEIFIKGKGFANASSVEHYLSDVCYTRAAELFKNAAIASGLRGKVKSNFRLKELKNMKSGLPTTKSDNFPIPLVKQKGGQYTGFEISSHNDDFIIKIPFGRWQVKKEINKFRPWEKFDFEQVRKSPKPISLLLSTQRRKRNKGWSRDEGTEAEIRKVMNGDYQTSYIEVKRGSKIGEKSAWMLNLSIDVPKIDKGVDPSIIGGIDVGVKSPLVCAINNAFSRYSISDNDLFHFNKKMFARRRILLKKTRHKRAGHGAKNKLKPISILTEKSERFRKKLIERWACEIADFFIKNRVGTVQMENLESMKRREDSYFNIRLRGFWPYAKMQNKIEFKLKQYGIEIRKVAPNNTSKTCSKCGHLNNYFNFEYRKKNKFPHFKCEKCNFKESADYNAALNISNPKLKSTKEEP

SEQ ID NO: 1678 - protein, 726 aa, synthetic construct
SEVEFSHEYWMRHALTLAKRARDKREVPVGAILVLNNRVIGEGWNRAIGLHDPTAHAEIMALRQGGLVMQNYRLIDATLYVTFEPCVMCAGAMIHSRIGRVVFGVRNNKHGAAGSLVNVLNYPGMNHRVEITEGILADECAALLCDFYRMPRQVFNARKKAQSSINSGGSSGGCSGSEMPGASESVTPKSSGGSSAGSTKNTITKTLKLRIVRPYNSAEVEKIVADEKNSREKIALERNKDKVKEACSEHLKVAAYCTTQVERNACLFCKARKLDDRFYQKLRGQFPDAVFWQETGEIFRQLQRQAAEIYNQSLIELYYEIFIKGKGFANASSVEHYLSDVCYTRAAELFKNAAIASGLRGKVKSNFRLKELKNMKSGLPTTKSDNFPIPLVKQKGGQYTGFEISSHNDDFIIKIPFGRWQMKKEIDKYRPWEKFDFEQVRKSPKPISLLLSTQRRKRNKGWSKDEGTEAEIRKVMNGDYQTSYIEVKRGSKIGEKSAWMLSLSIDVPKIDKGVDPSIIGGIDVGVKSPLVCAINDAFSRYSISDNDLFHFNKKMFARRRILLKKNRHKRAGHGAKNKRKPISILTEKNERFRKKLIERWACEIADFFIKNKVGTVQMENLESMKRKEDSYFNIRLRGFWPYAEMQNKIEFKLKQYGIEIRKVAPANTSKTCSKCGHLNNYFNFEYRKKNKFPHFKCEKCNFKENADYNAALNISNPKLKSTKEEP

SEQ ID NO: 1679 - protein, 726 aa, synthetic construct
SEVEFSHEYWMRHALTLAKRARDEREVPVGAVLVLNNRVIGEGWNRAIGLHDPTAHAEIMALRQGGLVMQNYRLIDATLYVTFEPCVMCAGAMVHSRIGRVVFGVRNSKRGAAGSLMNVLNYPGMDHRVEITGGILADECAALLCDFYRMPRRVFNAQRKAHSSINSGGSSGGSSGSVTPGTSESATPESSGGGFGDSAKNTITKTLQLRIVRPYNSAEVEKIVADEKNNREKIALEKNKDKVKEACSKHLKVASYCTTQVERNACLFCKARKLDDKFYQKLRGQFPDAVFWQELGEIFRQLQKQAAEIYNQSLIELYYEIFIKGKGLANASSVEHYLSDVCYTRAAELFKNAAIASGLRGKVKSNFKLKELKSMKSGLPSTKSDNFPIPLVKQKGGQYTGFEISSHNNDLIIKIPFGRWQVKREIDKYRPWEKFDFEQVRKSPKPISLLLSTQRRKRNKGWSKDEGTEAEIRKVMNGDYQTSYIEVKRGSKIGEKSAWMLNLSIDVPKIDKGVDPSIIGGIDVGVKSPLVCAINNALSRYSISDNDLFHFNKKMFARRRILLRKNRHKRAGHGAKNKLKPITIMTEKSKRFRKKLIERWACEIADFFIKNKVGTVQMENLESMKRKEDSYFNVRLRGFWPYAEMQNKIEFKLKQYGIKIRKVAPNNTSKTCSKCGHLNNYFSFEYRKKNKFPHFKCEKCNFREDADYNAALNISNPKLKSTKEDP

SEQ ID NO: 1680 - protein, 726 aa, synthetic construct
SEVEFSHEYWMRHALTLAKRARDEREVPVGAVLVLNNRVIGEGWNRAIGLHDPTAHAEIMALRQGGLVMQNYRLVDATLYVTFEPCVLCAGAMVHSRIGRVVFGVRNSKRGAAGSLMNVLNHPGMNHRVEITEGILADECAALLCDFYRMPRQVFNAQKKARSNINSGGSSGGSSGSETPGTSESATPVSSSGSSGGPAKNTITKTLKLRIVRPYNSAEVEKIVADEKNNREKIALEKNKDKVKEACSEHLKVAAYCTTQVERNACLFCKARKLDDKFYQKLRGQFPDAVSWQEIGEIFRQLQRQAAEIYNQSLIELYYEIFIKGKGFANASSVEHYLSDVCYTRAAELFKNAAIASGLRGKVKSNFRLKELKNMKSGLPTTKSDNFPIPLVKQKGGQYTGFEISSHNDDFIIKIPFGRWQVKEGIDKYRPWEKFDFEQVRKNPKPISLLLSTQRRKRNKGWSKDEGTEAEIRKVMNGDYQTSYIEVKRGSKIGEKSAWMLNLSIDVPKVDKGVDPSIIGGIDVGVKSPLVCAINNAFSRYSISDNDLYRFNKKMFARRRILLKKSKHKRAGHGAKNKLKPITILTEKSGRFRKKLIERWACEIADFFIKNKVGTVQMENLESMKGKEDSYFNIRLRGFWPYAEMQNKIEFKLKQYGIEIRKVAPNNTSKTCSKCGHLNNYFNFEYRKKNKFPHFKCEKCYFKEDADYNAALNISNPRLKSTKEEP

SEQ ID NO: 1681 - protein, 726 aa, synthetic construct
SEVEFSHEYWMRHALTLAKRARDEREVPVGAILVLNNRVIGEGWNRAIGLHDPTAHAEIMALRQGGLVMQNYRLIDATLYVTFEPCVMCAGAMIHSRIGRVVFGARNSKHGAAGSLVNVLDYPGMNHRVEITEGILADECAALLCDFYRMPRQVFNARKKAQSSINSGGSSGGSSGSETPGASGSVTPKSSGGSSAGSTKDTITKTLKLRIVRPYNSAEVEKIVADEKNNREKIALERNKDKVKEACSEHLKVAAYCTTQVERNACLFCKARKLDDRFYQKLRGQFPDAAFWQEIGEIFRQLQKQAAEIYNQSLIELYYEIFIKGKGFANASSVEHYLSDVCYTRAAELFKNAAIASGLRGKVKSNFKLKELKNMKSGLPTTKSDNFPIPLVRQKGGQYTGFEISSHNDDFIIKIPFGRWQVRKEIDKYRPWEKFDFEQVRKSPKPISLLLSTQRRKRNKGWSKDEGTEAEIRKVMNGDYQTSYIEVKRGSKIGEKSAWMLNLSIDVPKIDKGVDPSIIGGIDVGVKSPLVCAINNAFSRYSISDNELFHFNKKMFARRRILLKKSRHKRAGHGAKNKLKPITMMTEKSKRFRKKLIERWACEIADFFIKNKVGTVQMENLEGMRRKEDSYFNIRLRGFWPYAEMQNKIEFKLKQYGIVVRKVAPNNTSKTCSKCGHLNNYFNFEYRKKNKFPHFKCEKCNFKENADYNAALNISDPKLKSTKKEP

SEQ ID NO: 1682 - protein, 726 aa, synthetic construct
SEVEFSHEYWMRHALTLAKRARDEREVPVGAILVLNNRVIGVGWNRAIGLHDPTAHAEIMALRQGGLVTQNYRLIDATLYVTFEPCVMCAGAMIHSRIGRVVFGVRNSKHGAAGSLVNVLNYPGMNHRVEITEGILADECAALLCDFYRMPRQVFNARKKAQSSVNSGGSSGGTSGSKTPVTSESATPESPGGSSGGSTKDTITKTLKLRIVRPYNSAEVEKIVADEKNNREKIALERNKGKVKEACSKHLKVATYCTTQVERNACLFCKARKLDDKFYQKLRGQFPDAVFWQEIGEIFRQLQKQAAEIYNQSLIELYYEIFIEGKGSANARSVEHYLSDVCYTRAAELFKNAAIASGLRGKVKSNFRLKELKNMKSGLPTTKSDNFPIPLVKQKGGQYTGFEISSHNDDFIIKIPFGRWQVKKEIDKYRPWEKFDFEQVRKSPKPISLLLSTQRRRRNKGWSKDEGTEAEIRKVMNGDYQTSYIEVKRGSKTGEKSAWMLNLSIDVPKIDKGVDPSIIGGVDVGVKSPLVCAINNAFSRYSISDNDLFRFNKKVFARRRILLKKNRHKRAGHGAKNKLKPISILTGKSERFRKKLIERWACEIADFFIKNKVGTVQMENLESMKRREDSYFNIRLRGFWPYAEMQNKIEFKLKQYGIEVRKVAPNNTSKTCSKCGHLNNYFNFEYRKKNKFPHFKCEKCNFKENADYNAALNISNPKLKSTKEEP

SEQ ID NO: 1683 - protein, 726 aa, synthetic construct
SEVEFSHEYWMRHALTLAKRARGEREVPVGAILVLNNRVIGEGWNRAIGLHDPTAHAEIMALRQGGLVMQNYRLTDATLYVTFEPCVMCAGAMIHSRIGRVVFGVRNNKHGAAGSLVNVLNYPGMNHRVEITEGILADECAALLCDFYRMPRQVFNARKKAQSSINPGGSSGGSSGSETPGTRESATPKNSGGSSGGSAKNTITKALKLRIVRPYNSAEVEKIVADEKNNRERIALEKNKDKVKEACSKHLKVAAYCTTQVERNACLFCKARKLDDKFYQKLRGQFPDAVFWQEIGEIFRQLQKQAAEIYNQSLIELYYEIFIKGKGFANASSVEHYLSDVCYTRAAELFKNAAIASGLRGKVKSNFRLKELKNMRSGLPTTKSDNFPIPLVKQKGGQYAGFEISSHNDDFIIKIPFGRWQVKKEIDKYRPWEKFDFEQVRRSPKPISLLLSTQRRKKNKGWSKDEGTEAEIRRVMNGDYRISYIEVKRGGKIGERSAWMLNLSIDVPKIDKGVDPSIIGGIDVGVKSPLVCAINNAFSRYSVSDNDLFHFNKKMFARRRILLKKNRHKRAGHGAKNKLKPITILTEKSERFRKKLIERWACEIADFFIKNKVGTVQMEDLESMKGKEDSYFNIRLRGFWPYAEMQNKIEFKLKQYGIEIRKVAPNNTSKTCSKCGHLNSYFNFEYRKKNKFPHFKCEKCNFKENADYNAALNISNPKLKSTKEEP

SEQ ID NO: 1684 - protein, 726 aa, synthetic construct
SEVEFSHEYWMRHALTLAKRARDEREVPVGAILVLNNRVIGEGWNRAIGLHDPTAHAEIMALRQGGLVTQNYRLIDATLYVTFEPCVMCAGAMIHSRIGRVVFGVRNNKHGAAGSLVNVLNYPGMNHRVEITEGILADECAALLCDFYRMPRQVFNARKKAQSSINPGGSSGGSSGSETPGTSGSATPESSGGSSGGSAKNTITKTLKLRIVRPYNSAEVEKIVADEKDSREKIALEKNRNKVKEACSKHLKVAAYCTTQVERNACLFCKARRLDDKFYQKLRGQFPDAVFWQEIGEIFRQLQKQAAEVYNQSLVELYYEIFIKGKGIANASSVEHYLSDVCYTRAAELFKNAAIASGLRNKIKSNFRLKELRNMKSGLPTTKSDNFPIPLVRQKGGQYTGFEISNHDGDFIIKIPFGRWQVKKEINKHRPWEKFDFEQVRKSPKPISLLLSTRRRKRNKGWSKDEGTEAEIRKVMNGDYQTSYIEVKRGSKIGEKSAWMLNLSIDVPKIDKGVDPSIIGGIDVGVKSPLVCAINNAFSRYSISDNDLFRFNKKMFARRRILLRKNRHKRAGHGAKNKLKPITMMTEKSKRFRKKLIERWACEIADFFIKNKVGTVQMENLESMKRKEDSYFNIRLRGFWPYAEMQNKIEFKLKQYGIVVRKVAPNNTSKTCSKCGHLNNYFDFEYRRKNKFPLFKCEKCSFKENADYNAALNISNPKLKSTKGEP

SEQ ID NO: 1685 - protein, 726 aa, synthetic construct
SEVEFSHEYWMRHALTLARRARDEREVPVGAILVLNNRVIGEGWNRAIGLNDPTAHAEIMALRQGGLVMQNYRLIDATLYVTFEPCVMCAGAMIHSRIGRVVFGVRNNKHGAAGSLMNVLNYPGMNHRVEITEGILADECAALLCDFYRMPRQVFNARKKAQSSINPGGSSGGSGGSETPGTSESATPENSGGSSGSSAKNTITKTLKLRIVRPYNSAEVEKIVADEKNNRERIALEKNKDKVKEACSKHLKVASYCTTQVERNACLFCKARKLDDKFYQKLRGQFPDAVFWQELGEIFRQLQKQAAEIYNQSLIELYYVIFIKGKGLANASSVEHYLSGVCYTRAAELFKNAAIASGLRGKVKSNFRLKELKNMKSGLPTTKSDNFPIPLVKQKGGQYTGFEISSHNDDLIVKIPFGRWQVKKEIDRYRPWEKFDFEQVRKSPKPISLLLSTQRRKRNKGWSKDEGTEAEIRKVMNGDYQTSYIEVRRGSKIGEKNAWMLSLSIDVPKIDKGVDPSIIGGIDVGVKSPLVCAINNACSRYSISDNDLFHFNKKMFARRRILLKKNGHKRAGHGAKNKLRPITIMTEKSKRFRKKLIERWACEIADFFIKNKVGAVQMENLESMRRKEDSYFNIRLRGFWPYAEMQNKIEFKLKQYGIVVRKVAPNNTSKTCSKCGHLNNYFNFEYRKKNKFPHFKCEKCNFKENADYNAALNISDPKLKSTKKEP

SEQ ID NO: 1686 - protein, 726 aa, synthetic construct
SEVEFSHEYWMRHALTLAKRARDEREVPVGAVLVLNNRVIGVGWNRAIGLHDPTAHAEIMALRQGGLVMQNYRLTDATLYVTFEPCVMCAGAMIHSRIGRVVFGVRNSKRGAAGSLMNVLNYPGMNHCVEITEGILVDECAALLCDFYRMPRQVLNAQKKAQSSISSGGSSGGSSCSETPGASESVTPKSSGGGSAGSTKNTITKTLKLRIVRPYNSAEVEKIVADEKNSREKIALEKNKDKVKEACSEHLKVAAYCTTQVERNACLFCKARKLDDRFYQKLRGQFPDAVFWQEIGEIFRQLQKQAAEIYNQSLIELYYEIFIKGKGFANASSVEHYLSDVCYTRAAELFKNAAIASGLRGKVKSNFRLKELKSMKSGLPTTKSDNFPIPLVKQKGGQYTGFEVSSHNDDFIIKIPFGRWQVKKEIDKYRPWEKFDFEQVRKSPRPISLLLSTRRRKRNKGWSKDEGTEAEIRKVMNGDYQTSYIEVKRGSRIGEKSAWMLNLTIDVPKIDKGVDPSIIGGIDVGVKSPLVCAIDNAFSRYSISDNDLYHFNKKMFAKRRILLKKNRHKRAGHGAKNKLKPISILTEKSERFRRKLIERWASEIADFFIKNKVGTVQMENLESMKRREDSYFNTRLRGFWPYAEMQNKIEFKLKQYGIEIRKVAPNNTSKTCSKCGHLNNYFNFEYRKKNKFPHFKCEKCNFKEDADYNAALNISNPKLKSTKEES

SEQ ID NO: 1687 - protein, 726 aa, synthetic construct
SEVEYSHEYWMRHALTLAKRARDEREVPVGAILVLNNRVIGVGWNRAIGLHDPTAHAEIMALRQGGLVMQNYRLIDATLYVTFEPCVMCAGAMIHSRIGRVVFGVRNSKHGAAGSLVNVLNYPGMNHRVEITEGILADECAALLCDFYRMPRQVFNARKKAQSSINSGGSSGGSSGSETPGTSESATPKSSGGSSGGSAKNTITKALKLRIVRPYNSAEVEKIVADEKNNRERIALEKNKDKVKEACSKHLKVAAYCTTQVERNACLFCKARRLDDKFYQKLRGQFPDAVFWQEIGEIFRQLQKQAAEVYNQSLVELYYEILIKGKGIANASSVEHYLSDVCYTRAAELFKNAAIASGLRNKIKSNFRLKELRNMKSGLPTTKSDNFPIPLVRQKGGQYTGFEISNYNGDFIIKIPFGRWQVKKEINKHRPWEKFDFEQVRKSPKPISLLLSTQRRKRNKGWSKDEGTEAEIRKAMNGDYQTSYIEVKRGSKIGEKSAWMLSLSIDVPKIDKGVDPRIIGGIDVGVKSPLVCAINNVLSRYSISDNDLFHFNKKMFARRRILLKKNGHKRAGHGAKNKLKPITIMTEKSKRFRKKLIERWACEIADFFIKNKVGTVQMENLESMKRKEDSYFNIRLRGFWPYAEMQNKIEFKLKQYGIEIRKVAPNNTSKTCSKCGHLNNYFNFEYRKRNKFPHFKCEKCNYKEDADYNAALNISNPKLKSTKEEP

SEQ ID NO: 1688 - protein, 726 aa, synthetic construct
SEVEFSHEYWMRHALTLAKRARDEREVPVGAVLVLNNRVIGEGWNRAIGLHDPTAHAEIMALRQGGLVMQNYRLIDATLYVTFEPCVMCAGAMVHSRIGRVVFGVRNSKRGAAGSLMNVLDYPGMGHRVEITEGILADECAALLCDFYCMPRRVFNAQKRAQSSINSGGSSGGSGGGETPGASESVTPKSFGGSSAGSTKNTITKTLKLRIVRPYNSAEVEKIVADEKNNREKIALEKNKDKVKEACSKHLKVAAYCTTQVERNACLFCKARRLDDKFYQKLRGQFPDAVFWQEIGEIFRQLQKQAAEVYNQSLVELYYEILIKGKGIANASSVEHYLSDVCYTRAAELFKNAAIASGLRGKVKSNFRLKELKNMRSGLPTTKSDNFPIPLVKQKGGQYAGFEISSHNDDFIIKIPFGRWQVKKEIDKYRPWEKFDFEQVRKSPKPISLLLSTRRRKRNRGWSKDEGTEAEIRKVMNGDYQTSYIEVKRGSKIGEKSAWMLNLSIDVPKIDKGVDPSIIGGIDVGVKSPLVCAINNAFSRYSISDNDLFCFNKKMFARRRILLGKNRHKRAGHGVKNKLKPITILTEKSGRFRKKLIERWACEIADFFVKNKVGTVQMENLESMKRKEDSYFNIRLRGFWPYAEMQNKIEFKLKQYGIEIRKVAPNNTSKTCSKCGHLNNYFNFEYRKKNKFPHFKCEKCNFKENADYNAALNISNPKLKSTKEEP

SEQ ID NO: 1689 - protein, 726 aa, synthetic construct
SEVEFSHEYWMRHALTLAKRARDGREVPVGAVLVLNNRVIGEGWNRAIGLHDPTAHAEIMALRQGGLVMQNYRLIDATLYVTFEPCVMCAGAMVHSRIGRVVFGVRNSKRGAAGSLMNVLDYPGMGHRVEITEGILADECAALLCDFYCMPRRVFNAQKRAQSSINSGGSSGGSSGSETPGTSESATPESSGGGSSGSAKNTITKTLQLRIVRPYNSAEVEKIVTDEKNNREKIALEKNKDKVKEACSKHLKMASYCTTQVERNACLFCKARKLDDKFYQKLRGQFPDAVFWQELGGIFRQLQKQAAEIYNQSLIELYYEIFIKGKGITNASRVEHYLSDVCYTRAAELFKNAAIASGLRSKVRSNFRLKELKNMKSGLPTTKSDNFPIPLVKQKGGQYTGFEISSHNSDFIIKIPFGRWQVKEEIDKYRPWEKFDFEQVRKSPKPISLLLSTQRRKRNKGWSKDEGTEAEVRKVMNGDYRTSYIEVKRGSKIGEKSAWMLNLSIDVPKIDKGVDPSIIGGIDVGVKSPLVCAINNSSSRYSICDNDLFRFNKKMFARRRILLKKNRHKRAGHGAKNKLKPITILTKKSERFRKKLIERWVCEVADFFIKNKVGTVQMENLESMKRKEDSYFNIRLRGFWPYAEMQNRIELKLKQYGIEIRRVAPNNTSRTCSKCGHLNNYFNFEYRKKSKFPHFKCEKCNFREDADYNAALNISNPKLKSTKEEP

SEQ ID NO: 1690 - protein, 725 aa, synthetic construct
SEVEFSHEYWMRHALTLAKRARDEREVPVGAVLVLNNRVIGEGWNRAIGLHDPTAHAEIMALRQGGLAMQNYRLVDATLYVTFEPCVLCAGAMVHSRIGRVVFGVRNSKRGAAGSLMNVLNYPGMNHRVEITEGILADECAALLCDFYRMPRQVFNAQKKARPNINSGGSSGGRSGSETPGTSESATPESSGGSSGGSAKNTITKTLKLRIVRPYNSAEVEKIVADEKNNREKVALEKNKDKVKEACSKHLKVAAYCTTQVERNACLFCKARKLDDKFYQKLRGQFPDAVFWQELGEILRQLQKQAAEIYNQSLIELYYEIFIKGRGFANASSVEHYLSDVCYTRAAELFKNAAIASGLRSKVRSNFRLKELKNMRSGLPTTKSDNFPIPLVKQKGGQYTGFEISSHNDDFIIKIPFGRWQVKKEINKYRPWEKFDFEQVRRNPKPISLLLSTQRRKRNKGWSKDEGTEAEIRKVMNGDYRTSYIEVKRGSKTGEKSAWMLNLSIDVPKIDKGVDPSIIGGIDVGVKSPLVCAINNAFSRYSISDNDLFRFNKKMFARRRILLKKNRHKRAGHGAKNKLKPISILTGKSERFRKKLIERWACEIADFFIKNKVGTVQMENLESMKRKEDSYFNIRLRGFWPYAEMNRIEFKLKQYGIEIRKVAPNNTSKTCSKCGHLNNYFNFEYRKKNKFPHFKCEKCNFKENADYNAALNISNPKLKSTKERP

SEQ ID NO: 1691 - protein, 726 aa, synthetic construct
SEVEFSHEYWMRHALTLAKRARDEREVPVGAILVLNNRVIGEGWNRAIGLHDPTAHAEIMALRQGGLVMQNYRLIDATLYVTFEPCVMCAGAMVHSRIGRVVYGVRNSKRGAAGSLMNVLDYPGMDHRVEITEGILADECAALLCDFYRMPRQVFNAQKKAQSSINSGGSSGGSSGSETPGTSESTTPESSGGSSGGSARNTITKTLQLRIVRPYNSAEVEKIVADEKNRREKIALEKNKDKVKEACSKHLMVASYCTTQVERNACLFCKARELDGKFYQKLRGQFPDAVFWQELGEIFRQLQKQAAEIYNQSLIELYYEIFVKGKGIANTSRMEHYLSDVCYTRAAKLFKNAAIASGLRGKIKSNFRLKELKSMKSGLPTTRSDNFPIPLVKQKGGQYTGFEISNHDSDFIIKIPFGRWQVKKEIDKYRPWEKFDFEQVRKSPKPISLLLSTQRRRRNKGWSKDEGTEAEIKKVMNGDYQTSYIEVKRGSKIGEKSAWMLNLSIDVPKIDKGVDPSIIGGIDVGVKSPLVCAINNACSRYSISDNDLFHFNKKMFARRRILLKKNRHKRAGHGAKNKLKPLTILTGKSKRFRKKLIERWACEIADFFIKNKVGTVQMEDLESMKRKEDSYFNTRLRGFWPYAEMQNKIEFKLKQYGIEIRKVAPNNTSKTCSKCGHLNNYFNFEYRKRNKFPRFKCEKCNFKENADYNAALNISNPKLKGPKEES

SEQ ID NO: 1692 - protein, 726 aa, synthetic construct
SEVEFSHEYWMRHALTLAKRARDEREVPVGAVLVLNNRVIGEGWNRAIGLHDPTAHAEIMALRQGGLVMQNYRLVDATLYVTFEPCVLCAGAMVHSRIGRVVFGVRNNKRGAAGSLMNVLDYPGMNHRVEITEGILADECAALLCDFYRMPRQVFNAQKKARPNINSGGSSGGSSGSVTPGTSESATPESSGGGFGGSAKNTITKTLQLRIVRPYNSAEVEKIVANEKNNREKIALEKNKDKVKEACSKHLKVASYCTTQVERNACLFCKARKLDDKFYQKLRDQFPDAVFWQELGEIFRQLQKQAAEIYNQSLIELYYEIFIKGKGLANASSVEHYLSDVCYTRAAELFKNAAIASGLRGKVKSNFKLKELKSMKSGLPSTKSDNFPIPLVKQRGGRYTGFEISSHNDDFIIKIPFGRWQAKKEIDKYRPWEKFDFEQVRKSPKPISLLLSTQRRKRNRGWSKDEGTEAEIRKVMNGDYQTSYIEVKRGSKFGEKSAWMLNLSIDVPKIDKGVDPSIIGGIDVGVKSPLVCAINNAFSRYSISDNDLFRFNKKMFARRRILLGKNRHKRAGHGVKNKLKPITILTEKSGRFRKKLIERWACEIADFFIKNKVGTVQMENLESMKRKEDSYFNIRLRGFWPYAEMQNKIEFKLKQYGIEIRRVAPNNTSKTCSKCGHLNNYFNFEYRKKNKFPHFKCEKCNFKENADYNAALNISNPKLKSTKEEP

SEQ ID NO: 1693 - protein, 726 aa, synthetic construct
SEVEFSHEYWMRHALTLAKRARDECEVPVGAVLVLNNRVIGEGWNRAIGLHDPTAHAEIMALRQGGLVMRNYRLTDATLYVTFEPCVMCAGAMIHSRIGRVVFGVRNSKRGAAGSLMNVLNYPGMNHCVEITEGILVDECAALLCDFYRMPRQVLNAQKKARSNINSGGSSGGSSGSETLGTSESATPESSGGSSGGSAKNTITKTLKLRIVRPYNSAEVEKIVADEKNNREKIALEKNKDKVKEACSEHLKVAAYCTTQVERNACLFCKARKLDDKFYQKLRGQFPDAVFWQEISEIFRQLQKQAAEIYNQSLIELYYEIFIKGKGFANASSVEHYLSDVCYTRAAELFKNAAIASGLRGKVKSNFRLKELKSMKSGLPTTKSDNFPIPLVKQKGGQYTGFEISSHNDDFIIKVPFGRWQVKKEIDKYRPWEKFDFEQVRKSPKPISLLLSTQRRKRNKGWSKDEGTEAEIRRVMNGDYQTSYIEVKRGSKIGEKSAWMLNLSIDVPKIDKGVDPSIIGGIDVGVKSPLVCAINNAFSRYSISDNDLFHFNKKMFARRRILLKKSKHKRAGHGAKSKLKPITILTEKSGRFRKKLIERWACEIADFFIKNKVGTVQMENLESMKRKEDSYFNIRLRGFWPYAEMQNKIEFKLKQYGIEIRKVAPNNTSKTCSKCGHLNNYFNFEYRKKNKFPHFRCEKCNFKENADYNAALNISNPKLKSTKEEP

SEQ ID NO: 1694 - protein, 726 aa, synthetic construct; identical to SEQ ID NO: 684

SEQ ID NO: 1695 - protein, 726 aa, synthetic construct
SEVEFSHEYWMRHALTLAKRARDEREVPVGAVLVLNNRVIGEGWNRAIGLHDPTAHAEIMALRQGGLVMQNYRLIDATLYVTFEPCVMCAGAMVHSRIGRVVFGVRNSKRGAAGSLMNVLDYPGMGHRVEITEGILADECAALLCDFYCMPRQVFNAQKRAQSSINSGGSSGGSSGSETPGTSESATPESSGGGSSGSAKNTITKTLQLRIVRPYNSAEVEKIVADEKNNREKIALEKNKDKVKEACSKHLKVASYCTTQVERNACLFCKARKLDDKFYQKLRGQFPDAVFWQELGGIFRQLQKQAAEIYNQSLIELYYEIFIKGKGITNASRVEHYLSDVCYTRAAELFKNAAIASGLRSKVRSNFRPKELKNMKSGLPTTKSDNFPIPLVKQKGGQYTGFEISSHNSDFIIKIPFGRWQEKEEIDKYRPWEKFDFEQVRRSPKPISLLLSTQRRKKNKGWSKDEGTEAEIRRVMNGDYQTSYIEVKRGSKIGEKSAWMLSLSIDVPKIDKGVDPSIIGGVDVGVKSPLVCAINNAFSRYSISDNDLFHFNKKMFARRRILLKKNRHKRAGHGAKNKLKPISILTGKSERFRKKLIERWACEIADFFIKNKVGTVQMENLESMKRKEDSYFNIRLRGFWPYAEMQNKIEFKLKQYGIEIRKVAPNNTSKTCSKCGHLNNYFNFEYRRKNKFPHFKCEKCNFKENADYNAALNISNPKLKSTKEEP

SEQ ID NO: 1696 - protein, 726 aa, synthetic construct
SEVEFSHEYWMRHALTLAKRARDEREVPVGAVLVLNNRVIGEGWNRAIGLHDPTAHAEIMALRQGGLVMQNYRLIDATLYVTFEPCVMCAGAMVHSRIGRVVFGVRNSKRGAAGSLMNVLDYPGMGHRVEITEGILADECAALLCDFYCMPRQVFNAQKKAQSSISSGGSSGGCSGSEMPGASESVTPKSSGGSSAGSTKNTITKTLKLRIVRPYNSAEVEKIVADEKNSREKIALERNKDKVKEACSEHLKVAAYCTTQVERSACLFCKARKLDDKFYQKLRDQFPDAVFWQEIGEIFRQLQRQAAEIYNQSLIELYYEIFIKGKGFANASSVEHYLSDVCYTRAAELFKNAAIASGLRGKVKSNFRLKELKNMKSGLPTTKSDNFPIPLVKQKGGQYTGFEISSHNDDFIIKIPFGRWQVKKEIDKYRPWEKFDFEQVRKSPKPISLLLSTRRRKRNKGWSKDEGTEAEIRKVMNGDYQTSYIEVKRGSKIGEKSVWMLNLSIDVPKIDKGVDPSIIGGIDVGVKSPLVCAINNAFCRYSISDNDLFHFNKKMFARRRILLKKSRHKRAGHGAKNKLKPITILTEKSVRFRKKLIERWACEIADFFIKNKVGTVQMENLESMKRKEDSYFNIRLRGFWPYAEMQNKIEFKLKQYGVEIRRVAPNNTSRTCSKCGHLNNYFNFEYRRKNKFPHFKCEKCNFKEDADYNAALNISNPKLKSTREEP

SEQ ID NO: 1697 - protein, 726 aa, synthetic construct
SEDEFSHEYWMRHALTLAKRARDGREVPVGAVLVLNNRVIGEGWNRAIGLHDPTAHAEIMALRQGGLVMQNYRLIDATLYVTFEPCVMCAGAMVHSRVGRVVFGVRNSKRGAAGSLMNVLDYPGMGHRVEITEGILADECAALLCDFYCMPRQVFNAQKRAQSSINPGGSSGGSSGSETPGTSESATPGSSGGGSSGSTKNTITKTLKLRIVRPYNSAEVEKIVADEKNNREKIALEKNKDKVREACSKHLKVAAYCTTQVERNACLFCKARKLDDKFYQKLRGQFPDAVFWQEIGEIFRQLQKQAAEIYNQSLIELYYEIFIKGKGFASASSVEHYLSDVCYTRAAELFKNAAIASGLRGKVKSNFRLKELKNMKSGLPTTRSDNFPIPLVRQKGGQYTGFEISSHNDDFIIKIPFGRWQVKEEIDKYRPWEKFDFEQVRRNPKPISLLLSTQRRKRNKGWSKDEGTEAEIRKVMNGDYQTSYIEVKRGSKIGEKSAWMLNLSIDVPKIDKGVDPSITGGIDVGVKSPLVCAINNAFSRYSISDNDLFHFNKKMFARRRILLKKNRHKRAGHGAKNKLKPISILTEKSKRFRKKLIERWACEIADFFIKNKVGTVQMENLESMKRKEDSYFNIRLRGFWPYAEMQNKIEFKLKQYGIEIRKVAPNNTSKTCSKCGHLNNYFNFEYRKMNKFPHFKCEKCNFKENADYNAALNISNPKLKSTKEEP

SEQ ID NO: 1698 - protein, 726 aa, synthetic construct
NEVEFSHEYWMRHALTLAKRARDEREVPVGAVLVLNNRVIGEGWNRTTGLHDPTAHAEIMALRQGGLVMQNHRLVDATLYVTFEPCVMCAGAMIHSRIGRVVFGVRNSKHGAAGSLVNVLNYPGMNHRVEITEGILADECAALLCDFYRMPRQVFNARKKAQSSINSGGSSGGSGGSETPGTSESATLENSGGSSGGSAKNTITKTLKLRIVRPYNSAEVEKIVADEKDSREKIALEKNKDKVTEACSEHLKVATYCTTQVERNACLFCKARKLDDKFYQKLRGQFPDAVFWQEIGEIFRQLQKQAAEIYNQSLIELYYEIFIKGKGFANASSVEHYLSDVCYTRAAELFKNAAIASGLRNKTKSNFRLKELRSMKSGLPTTKSDNFPIPLVKQKGGQYTGFEISNHNSDFIIKIPFGRWQAKKEIDKYRPWEKFDFEQVRKSPKPISLLLSTQRRKRNKGWSKDEGTEAEIEKVMNGDYQTSYIEVKRGSKTGGKSAWMLNLSIDVPKIDKGVDPCIIGGIDVGVKSPLVCAINDAFSRYSISDNDLFHFNKKMFARRRILLKKNGHKRAGHGAKNKLKPITIMTEKSKRFRKKLIERWASEIADFFIKNKVGTVQMENLESMKRREDSYFNIRLRGFWPYAEMQNKIEFKLKQYGIEIRKVAPNNTSKTCSKCGHLNNYFNFEFRKKNKFPHFKCEKCNFKENADYNAALNISNPKLKSTKEEP

SEQ ID NO: 1699 - protein, 726 aa, synthetic construct
SEVEFSHEYWMRHALTLAKRARDEREVPVGAVLVLNNRVIGEGWNRTTGLHDPTAHAEIMALRQGGLAMRNYRLVDATLYVTFEPCVLCAGAMVHSRIGRVVFGVRNSKRGAAGSLMNVLNHPGMNHRVEITGGILADECAALLCDFYRMPRQVFNARKKAQSSISPGGSSGGSSGSETPGTSESAAPKSSGGSSGGSAKNTITKTLKLRIVRPYNSAEVEKIVADEKNNREKIALEKNKDKVKEACSKHLKVAAYCTTRVERNACLFCKARRLDDKFYQKLRGQFPDAVFWQELGEILRQLQKQAAEIYNQSLIELYYEIFIKGRGFANASSVEHYLSNVCYTRAAELFKNAAIASGLRGKVKSNFRLKELKNMKSGLPTTKSDNFPIPLVKQKGGQYTGFEISSHNDDFIIKIPFGRWQVKREIDKYRPWEKFDFEQVRKSPKPISLLLSTQRRKRNKGWSKDEGTEAEIRKVMNGDYQTSYIEVKRGSKTGEKSAWMLNLSIDVPKIDKGVDPSIIGGIDVGVKSPLVCAISNAFSRYSISDNDLFHFNKKMFARRRILLKKSKHKRAGHGVKNKLKPITILTEKSRRFRKKLIERWACEIADFFIKNKVGTVQMENLEGMKRKEDSYFNIRLRGFWPYAEMQNKIELKLKQYGIEIRKVAPNNTSKTCSKCGHLNNYFNFEYRKKNKFPHFKCEKCSFKENADYNAALNISNPKLKSTKGEP

SEQ ID NO: 1700 - protein, 726 aa, synthetic construct
SEVEFSHEYWMRHALTLAKRARDEREVPVGAVLVLNNRVIGVGWNRAAGLHDPTAHAEIMALRQGGLVMQNYRLTDATLYVTFEPCVLCAGAMVHSRIGRVVFGVRNSKRGAAGSLMNVLNYPGMNHRVEITEGVLADECAALLCDFYRMPRRVFNAQKKAQSSINSGGSSGGGSGSETPSTSESTTPESSGGSSGGPAKNTITKTLKLRIVRPYNSAEVEKIVADEKNNREKIALEKNKDKVKEACSKHLKVASYCTTQVERNACLFCKARKLDDKFYQKLRGQFPDAVFWQELGEIFRQLQKQAAEIYNQSLIELYYEIFIKGKGFANAGSVEHYLSDVCYTRAAELFKNAAIASGLRGKVKSNFRLKELKNMKSGLPTTKSDNFPIPLVKQKGGQYTGFEISSHNDDFIIKIPFGRWQVKKEIDKYRPWEKFDFEQVRKSPKPISLLLSTQRRKRNKGWSKDEGTEAEIRKVMNGDYQTSYIEVKRGSKTGEKSAWMLNLSIDVPKIDKGVDPSIIGGIDVGVKSPLVCAINNAFSRYSISDNDLFRFNKKMFARRRILLKKNRHKRAGHGAKNKLKPISILTGKSERFRKKLIERWACEIADFFIKNKVGTVQMENLESMKRKEDNYFNIRLRGFWPYAEMQNKIEFKLKQYGIEIRKVAPNNTSKTCSKCGHLNNYFNFEYRKKNKFPHFKCERCSFKENADYNAALNISNPKLKSTKEEP

SEQ ID NO: 1701 - protein, 726 aa, synthetic construct
SEVEFSHEYWMRHALTLARRARDGREVPVGAVLVLNNRVIGEGWNRAIGLHDPTAHAEIMALRQGGLVMQNYRLIDATLYVTFEPCVMCAGAMIHSRIGRVVFGVRNSKHGAAGSLVNVLNYPGMNHRVEITEGILADECAALLCDFYRMPRQVFNARKKAQSSINPSGSSGGSSGSVTPGTSESATPESSGGGFGGSAKNTITKTLQLRIVRPYNSADVEKIVADEKNNREKIALEKNKDKVKEACSEHLKVAAYCTTQVERNACLFCKARKLDDKFYQKLRGQFPDAVFWQEIGEIFRQLQKQAAEIYNQSLIELYYEIFIKGKGFANASSVEHYLSDVCYTRAAELFKNAAIASGLRGKVKSNFRLKELKSMKSGLPTTKSDNFPIPLVKQKGGQYTGFEISSHNDDFIIKIPFGRWQMKKEVDKYRPWEKFDFEQVRKSPKPISLLLSTQRRKRNKGWSKDEGTEAEIRKVMNGDYQTSYIEVKRGSKIGEKSAWMLNLSIDVPKIDKGVDPSIIGGIDVGVKSPLVCAINNAFSRYSISDNDLFHFNKKMFARRRILLKKNGHRRAGHGAKNKLKPISVLTEKSKRFRKKLIERWACEIADFFIKNKVGTVQMENLESMKRKEDSYFNIRLRGFWPYAEMQNKIEFKLKQYGIEIRKVAPNNTSKTCSKCGHLNNYFDFEYRKKNKFPHFKCEKCNFKENADYNAALNISNPMLKSTKEEP

SEQ ID NO: 1702 - protein, 726 aa, synthetic construct
SEVEFSHEYWMRHALTLAKRARDEREVPVGAVLVLNNRVIGEGWNRAIGLHDPTAHAEIMALRQGGLVLQNYRLVDATLYVTFEPCVLCAGAMVHSRIGRVVFGARNSKRGAAGSLMNILNYPGMSHRVEITEGILADECAALLCDFYRMPRQVFNARKKAQSSINPGGSSGGSSGSETPGTSESATPESSGGSSGGSAKNTITKALKLRIVRPYNSAEVEKIVADEKNSREKIALEKNKDKVKEACSEHLKVAAYCTTQVERSACLFCKARKLDDRFYQKLRGQFPDAVFWQETGEIFRQLQRQAAEIYNQSLIELYYEIFIKGKGFANASSVEHYLSDVCYTRAAELFKNAAIASGLRGKVKSNFRLKELKNMKSGLPTTKSDNFPIPLVKQKGGQYTGFEISSHNDDFIIKIPFGRWQVKKEIDKYRPWEKFDFEQVRKSPKPISLLLSTQRRKRNKGWSKDEGTEAEIRKVMNGDYQTSYIEVKRGSKIGEKSAWMLSLSIDVPKIDKGVDPSIIGGIDVGVKSPLVCAINNAFCRYSISDNDLFHFNKRMFARRRILLKKSRHKRAGHGAKNKLKPISILTEKSKRFRKKLIERWACEIADFFIKNKVGTVQMENLESMKRKEDSYFNIRLRGFWPYAEMQNKIEFKLKQYGIEIRKVAPNNTSKTCSKCGHLNNYFSFEYRKKNKFPHFKCEKCNFKENADYNAALNISNPKLKSTKEGP

SEQ ID NO: 1703 - protein, 726 aa, synthetic construct
SEVEFSHEYWMRHALTLAKRARDEREVPVGAILVLNNRVIGEGWNRAIGLHDPTAHAEIMALRQGGLVMQNYRLTDATLYATFEPCVMCAGAMIHSRIGRVVFGVRNSKHGAAGSLMNVLNYPGMNHRVEITEGILADECAGLLCDFYRMPRQVFSARKKAQSSINPGGSSGDSSGGKAPGTSESATLESSGGSSGDSAKNSITKTLKLRIVRPYNSAEVEKIVADEKNNREKIALEKNKGKVEEACSKHLKVATYCTTQVERSACLFCKARKLDDKFYQKLRGQFPDAVFWQEIGEIFRQLQKQAAEIYNQSLIELYYEIFIKGKGFANASSVEHYLSDVCYTRAAELFKNAAIASGLRSKIKSNFRLKELRNMRGGLPTTKSDNFPIPLVKQKGGQYTGFEISSHNDDFIIKIPFGRWQVKKEIVKHRPWEKFDFEQVRKSPKPISLLLSTQRRKRNKGWSKDEGTEAEIRKVMNGDYQTSYIEVKRGSKIGEKSAWMLNLSIDVPKIDKGVDPSIIGGIDVGVKSPLVCAINNALSRYSISDNDLFHFNKKMFARRRILLRKNRHKRAGHGAKNKLKPITMMTEKSKRFRKKLIERWACEIADFFIKNKVGTVQMENLESMKRKEDSYFNIRLRGFWPYAEMQNKIEFKLKQYGIVVRKVAPNNTSKTCSKCGHLNNYFNFEYRKKNKFPHFKCEKCNFKEDADYNAALNISNPKLKSTKGEP

SEQ ID NO: 1704 - protein, 726 aa, synthetic construct
SEVEFSHEYWMRHALTLAKRARDEREVPVGAILVLNNRVIGEGWNRAIGLHDPTAHAEIMALRQGGLVMQNYRLTDATLYVTFEPCVMCAGAMIHSRIGRVVFGVRNSKHGAAGSLMNVLNYPGMNHRVEITEGILADECAALLCDFYRMPHRVFNGRKKAQSSINPGGSSGGSSGSETPGASGSVTPKSSGGSSAGSTKDTITKTLKLRIVRPYNSAEVEKIVADEKNSREKIALEKNKDKVKEACSEHLKVAAYCTTQVERNACLFCKARKLDDRFYQKLRGQFPDAVFWQEIGEIFRQLQKQAAEIYNQSLIELYYEIFIKGKGFANASSVEHYLSDVCYTRAAELFKNAAIASGLRGKVKSNFRLKELKNMKSGLPTTKSDNFPIPLVRQKGGQYTGFEISDHNGDFIIKIPFGMWQVKKEISKHRPWEKFDFEQVRKSPKPISLLLSTQRRKRNKGWSKDEGTEAEIRKVMNGDYQTSYIEVKRGSKIGEKSAWMLNLSIDVPKIDKGVDPSIIGGIDVGVKSPLVCAINNALSRYSISDNDLFHFNKKVFARRRILLKKNRHRRAGHGAKNKLKPITILTEKSKRFRKKLIERWACEIADFFIKNKVGTVQMENLESMKRKEDSYFNIRLRGFWPYAEMQNKIEFKLKQYGIEIRKVAPNNTSKTCSKCGHLNNYFNFEYRRKNKFPHFKCEKCNFKEDADYNAALNISNPKLKSTKEEP

SEQ ID NO: 1705 - protein, 726 aa, synthetic construct
SEVEFSHEYWMRHALTLAKRARDEREVPVGAVLVLNNRVIGEGWNRAIGLHDPTAHAEIMALRQGGLVMENYRLVDATLYVTFEPCVLCAGAMVHSRIGRVVFGVRNSKRGAAGSLMNVLNYPGMNHRVEITEGILADECAALLCDFYRMPRQVFNAQKKARSSINSGGSSGGSGDSETPGTSESATPESSGGSSGGSAKNTITKTLKLRIVRPYNSAEVEKIVADEKNNREKIALEKNKDKVKEACSKHLKVASYCTTQVERNACPFCKARKLDDKFYQKLRGQFPDAVFWQELGEILRQLQKQAAEIYNQSLIELYYEILIKGKGIANASRVEHYLSDVCYTRAAELFKNAAIASGLRSKIKSNFRLKELRNMKSGLPTTKSDNFPIPLVKQKGGQCTGFEISNHNSDFIIKIPFGRWQVKKEIDKYRPWEKFDFEQVRKSPKPISLLLSTQRRRRNKGWSKDEGTEAEIRKVMNGDYQTSYIEVKRGSKTGEKSAWMLNLSIDVPKIDKGVDPSIIGGIDVGVKSPLVCAINNAFSRYSISDNDLFRFNKKMFARRRILLKKSRHKRAGHGAKNKLKPITILTEKSRRFRKKLIERWASEIADFFIKNKVGTVQMENLESMKRKEDSYFNIKLRGFWPYAEMQNKIEFKLKQYGIEIRRVAPNNTSKTCSKCGHLNNYFNFEYRKKNKFPHFKCEKCSFKENADYNAALNVSNPKLKSTKEEP

SEQ ID NO: 1706 - protein, 726 aa, synthetic construct
SEVEFSHEYWMRHALTLAKRARDEREVPVGAVLVLNNRVIGEGWNRAIGLHDPTAHAEIMALHQGGLVMQNYRLIDATLYVTFEPCVMCAGAMIHSRIGRVVFGARNSKRGAAGSLMNVLSYPGMNHRVEITEGILADECAALLCDFYRMPRRVFNAQKKAQSSINSGGSSGGGSGSETPSTSESTTPESSGGSSGGPAKNTITKTLKLRIVRPYNSAEVEKIVADEKNNRERIALEKNKDKVKEACSKHLKVAAYCTTQVERNACLFCKARKLDDKFYQKLRGQFPDAVFWQEVGEIFRQLQKQAAEIYNQSLIELYYEIFIKGKGIANASSVEHYLSDVCYTRAAELFKNAAIASGLRNKIKSNFRLKELRNMKSGLPTTKSDNFPIPLVRQKGGQYTGFEISNHDGDFIIKIPFGRWQVKKEINKHRPWEKFDFEQVRKSPKPISLLLSTQRRKRNKGWSKDEGTEAEIRRVMNGDYQTSYIEVKRGSKIGEKSAWMLNLSIDVPKIDKGVDPSIIGGIDVGVKSPLVCAINNALSRYSISDNDLFHFNKKMFARRRILLRKNRHKRAGHGAKNKLKPITIMTEKSKRFRKKLIERWACEIADFFIKNKVGTVQMENLESMKRKEDSYFNIRLRGFWPYAEMQNKIEFKLKQYGIEIRKVAPNNTSKTCSKCGHLNYYFNFEYRKKNKFPHFKCEKCNFKEDADYNAALNISNPKLKSTKEEP

SEQ ID NO: 1707 - protein, 726 aa, synthetic construct
SEVEFSHEYWMRHALTLAKRARDEREVPVGAVLVLNNRVIGVGWNRAIGLHDPTAHAEIMALRQGGLVMQNYRLTDATLYVTFEPCVMCAGAMIHSRIGRVVFGVRNSKRGAAGSLMNVLNYPGMNHCVEITEGILVDECAALLCDFYRMPRQVLNAQKKAQSSISSGGSSGGSSCSETPGASESVTPKSSGGGSAGSTKNTITKTLKLRIVRPYNSAEVEKIVADEKNSREKIALEKNKGKVKEACSEHLKVAAYCTTQVERNACLFCKARKLDDRFYQKLRGQFPDAVFWQEIGEIFRQLQKQAAEIYNRSLIELYYEIFIKGKGFANASSVEHYLSDVCYTRAAELFKNAAIASGLRNKIKSNFRLKELRNMKSGLPTTKSDNFPIPLVKQKGGQYTGFEISSHNDDFIIKIPFGRWQVKKEIDKFRPWEKFDFEQVRKSPKPISLLLSTQRRKRNKGWSKDEGTEAEIRKVMNGDYQTSYIEVKRGSKIGEKSAWTLNLSIDVPKIDKGVDPSIIGGIDVGVKSPLVCAINNAFGRYSISDNDLFHYNKKMFARRRILQKKNRYKRAGHGAKNKLKPISILTEKSKRFRKKLIERWACEIADFFIKNKVGTVQIENLESMKRKEDSYFNIRLRGFWPYAEMQNKIEFKLKQYGIEIRKVAPNNTSKTCSKCGHLNSYFNFEYRKKNKFPHFKCERCNFRENADYNAALNISNPKLKSTKEEP

SEQ ID NO: 1708 - protein, 726 aa, synthetic construct
SEVEFSHEYWMRHALTLAKRARDEREVPVGAVLVLNNRVIGEGWNRAIGLHDPTAHAEIMALRQGGLVMQNYRLIDATLYVTFEPCVMCAGAMIHSRIGRVVFGVRNNKRGAAGSLMNVLNYPGMNHRVEITEGILADECAALLCDFYRMPHQVLNAQKKARSCINPGGSSGGSNGGETPGTSESATPGGSGVSSGGSTKNTITKTLKLRIVRPYNSAEVEKIVADEKNNREKIALEKNKDKVKEACSKHLKVAAYCTTQVERNACLFCKARKLDDKFYQKLRGQFPDAVFWQEVGEIFRQLQKQAAEIYNQSLIELYYEIFIKGKGFANASSVEHYLSDVCYTRAAELFKNAAIASGLRGKVKSNFRLKELKNMRSGLPTTKSDNFPIPLVKQKGGQYAGFEISSHNDDFIIKIPFGRWQVKKEIDKYRPWEKFDFEQVRKSPKPISLLLSTQRRKRNKGWSKDEGTEAEIRKVMNGDYQTSYIEVKRGSKIGEKSAWMLNLSIDVPKIDKGVDPSIIGGIDVGVRSPLVCAINNALSRYSVSDNDLFHFNKKMFARRRILLRKNRHKRAGHGAKNKLRPITTLTGKSERFRRKLIERWACEIADFFIKNKVGTVQMENLESMKRKEDNYFNIRLRGFWPYAEMQNKIEFKLKQYGIEIRKVAPNNTSKTCSKCGHLNNYFSFEYRKKNKFPHFKCEKCNFKEDADYNAALNISNPKLKSTKEEP

SEQ ID NO: 1709 - protein, 726 aa, synthetic construct
SEVEFSHEYWMRHALALAKRARGEREVPVGAVLVLNNRAIGEGWNRAIGLHDPTAHAEIMALRQGGLVMQNYRLTDATLYVTFEPCVLCAGAMVHSRIGRVVFGVRNSKRGAAGSLLNVLNYPGMNHRVEITEGILADECAALLCDFYRMPRQVFSAQKKAQSSINSGGSSGGSSGSKTPGTSESATPESSGGGSSGSAKNTITKTLQLRIVRPYNSAEVEKIVADEKNNREKIALEKNKDKVKEACSKHLKVASYCTTQVERNACPFCKARKLDDKFYQKLRGQFPDAVFWQELGEILRQLQRQAAEIYNQSLIELYYEIFIKGRGFANASSVEHYLSDVCYTRAAELFRNAAIASGLRGKVKSNFRLKELKNMKSGLPTTKSDNFPIPLVKQKGGQYTGFEISSHNDDFIIKIPFGRWQVKKEIDKYRPWEKFDFEQVRKSPKPISLLLSTQRRKRNKGWSKDEGTEAEIRKVMNGDYQTSYIEVKRGSKTGEKSAWMLNLSIDVPKIDKGVDPSIIGGIDVGVKSPLVCAINSAFSRYSISDNDLFRFNKKMFARRRILLKKNRHKRAGHGAKNKLKPISILTGKSERFRKKLIERWACEIADFFIKNKVGTVQMENLESMKRKEDSYFNIRLRGFWPYAEMQNKIEFKLKQYGIEIRKVAPNNTSKICSKCGHLNNYFNFEYRRKNKFPYFKCGKCNFKEDADYNAALNISNPKLKSTKEKP

SEQ ID NO: 1710 - protein, 726 aa, synthetic construct
SEVEFSHEYWMRHALTLAKRARDEREVPVGAVLVLNNRVIGGGWNRAIGLHDPTAHAEIMALRQGGLVMQSCRLVDATLYVTFEPCVMCAGAMIHSRIGRVVFGVRNSKRGAAGSLMNVLNYPGMNHRVEITEGILAGECAALLCDFYRMPRQVFNARKKAQSTINSGGSSGGSSSSETPGTSGSATPEGSGGSSGGSAKNTITKTLKLRIVRPYNSAEVEKIVADEKNNREKIALEKNKDKVKEACSKHLKVASYCTTQVERNACLFCKARKLDDKFYQKLRGQFPDAVFWQELGEIFRQLQKQAAEIYNQSLIELYYEIFIKGKGFANASSVEHYLSDVCYTRAAELFKNAAIASGLRGKVKSNFRLKELKNMKSGLPTTKSDNFPIPLVKQKGGQYTGFEISSHNDDFIIKIPFGRWQVKKEIDKYRPWEKFDFEQVRKSPKPISLLLSTQRRKRNKGWSKDEGTEAEIRKVMNGDYQTSYIEVKRGSKIGEKSAWMLNLSIDVPKIDKGVDPSIIGGIDVGVKSPLVCAINNAFSRYSIGDNDLFHYNKKVFARRRILLKKNRHKRAGHGAKNKLKPISILTEKSKRFRKKLIERWACEIADFFIKNKVGTVQMENLESMKRKEDSYFNIRLRGFWPYAEMQNKIEFKLKQYGVKIRRVAPNNTSRTCSKCGHLNNYFNFEYRRKNKFPHFKCEKCNFKEDADYNAALNISNPKLKSTREEP

SEQ ID NO: 1711 - protein, 726 aa, synthetic construct
SEDEFSHEYWMRHALTLAKRARDGREVPVGAVLVLNKRVIGEGWNRAIGLHDPTAHAEIMALRQGGLVMQNYRLIDATLYVTFEPCVMCAGAMVHSRIGRVVFGVRNSKRGAAGSLMNVLNYPGMGHRVEITEGILADECAALLCDFYCMPRQVFNAQKRAQSSINSGGSSGGSSGSETPGTSESATPESSGGSSGGSAKNTITKTLQLRIVRPYNSAEVEKIVADEKNNREKIALEKNKDKVKEACSKHLKVAAYCTTQVERNACLFCKARKLDDKFYQKLRGQFPDAVFWQEIGEIFRQLQKQAAEIYNQCLIELYYEIFIKGKGFANASSVEHYLSDVCYTRAAELFKNAAIASGLRGKVKSNFRLKELKNMKSGLPTTKSDNFPIPLVKQKGGQYTGFEISSHNDDFIIKIPFGRWQVKEEIDKYRPWEKFDFEQVRKNPKPISLLLSTQRRKRNKGWSKDEGTEAEIRKVMNGDYQTSYIEVKRGSKIGEKSAWMLNLSIDVPKVDKGVDPSIIGGIDVGVKSPLVCAINNAFSRYSISDNDLFHYNKKMFARRRILLKKNRHKRAGHGAKNKLKPISILTEKSKRFRKKLIERWACEIADFFIKNKVGTVQIENLESMKRKEDSYFNIRLRGFWPYAEMQNRIEFKLKQYGIEIRKVAPNNTSKTCSKCGHLNSYFNFEYRKKNKFPHFKCEKCNFRENADYNAALNISNPKLRSTKEEP

SEQ ID NO: 1712 - protein, 726 aa, synthetic construct
SEVEFSHEYWMRHALALAKRARDEREVPVGAILVLNNRVIGEGWNRAIGLHDPTAHAEIMALRQGGLVMQNYRLTDATLYATFEPCVMCAGAMIHSRIGRVVFGVRNNKHGAAGSLVNVLNYPGMNHRVEITEGVLADECAALLCDFYRMPRQVFNARKKAQSSINPGGPSGGSSGSKTPGTSESATPEGSGGGSSGSAKNTITKTLQLKIVRPYNSAEVEKIVADEKNNREKIALEKNKDKVKEACSKHLKVASYCTTQVERSACPFCKARKLDDKFYQKLGGQFPDAVFWQELGEILRQLQKQAAEIYNQSLIELYYEIFIKGRGFANASSVEHYLSDVCYTRAAELFKNAAIASGLRGKVKSNFRLKELKNMKSGLPTTKSDNFPIPLVKQKGGQYTGFEISSHNDDFIIKIPFGRWQVKKEIDKYRPWEKFDFGQVRRSPKPISLLLSTQRRKRNKGWSKDEGTEAEIRKVMNGDYQTSYIEVKRGSKTGEKSAWMLNLSIDVPKIDKGVDPNIIGGIDVGVKSPLVCAINNAFSRYSISDNDLFRFNKKMFARRRILLKKNRHRRAGHGAKNKLKPITILTEKSVRFRKKLIERWACEIADFFIKNKVGTVQMENLESMKRKEDSYFNIRLRGFWPYAEMQNKIEFKLKQYGIEIRKVAPNNTSKTCSKCGHLNNYFNFEYRKKNKFPHFKCEKCYFREDADYNAALNISNPKLRSTKEEP

SEQ ID NO: 1713 - protein, 726 aa, synthetic construct
SEVEFSHEYWMRHALTLAKRARDEREVPVGAILVLNNRVIGEGWNRAIGLHDPTAHAEIMALRQGGLVMQDYRLIDATLYVTFEPCVMCAGAMIHSRIGRVVFGVRNNKHGAAGSLVNVLNYPGMNHRVEITEGILAEECAALLCDFYRMPRQVFNARKKAQSSINPGGSSGGSSGSETPGTSESATPESSGGSSGGSAKNTITKTLKLRIVRPYNSVEVEKIVADEKNNREKIALEKNKDKVKEACSKHLKVAAYCTTQVERNACLFCKARKLDDKFYQKLRGRFPDAVFWQEISEIFRQLQKQAAEIYNQSLIELYYEIFIKGKGFANASSVEHYLSDVCYTRAAELFKNAAIASGLRGKVKSNFRLKELKNMKSGLPTTKSDNFPIPLVKQKGGQYTGFEISSHNDDFIIKIPFGRWQGKKEVDKYRPWEKFDFEQVRKSPKPISLLLSTRRRKRNKGWSKDEGTEAEIKKVMNGDYQTSYIEVKRGSKIGEKSAWMLSLSIDVPKIDRGVDPSIIGGIDVGVKSPLVCAINNASSRLSISDNDLFRFNKKMFARRRILLKKNGHKRAGHGAKNKLKPITILTEKSVRFRKKLIERWACEIADFFIRNKVGTVQMENLESMKRKEDGYFNIRLRGFWPYAEMQNKIEFKLKQYGIKIRKVAPNNTSKTCSKCGHLNNYFNFEYRKKNKFPHFKCEKCNFKENADYNAALNISNPKLKSTKGEP

SEQ ID NO: 1714 - protein, 726 aa, synthetic construct
SEVEFSHEYWMRHALTLAKRARDEREVPVGAVLVLNNRVIGEGWNRAIGLHDPTAHAEIMALRQGGLVMRNYRLTDATLYVTFEPCVMCAGAMIHSRIGRVVFGVRNSKRGAAGSLMNVLNYRGMGHRVEITEGILADECAALLCDFYCMPRQVFNAQKRAQSSINSGGSSGGSSGSETPGTSESPTPESSGGSSGGSAKNTITKTLKLRIVRPYNSAEVEKIVADEKSNREKIALEKNKDKVKEACSEHLKVAAYCTTQVERSACLFCKARKLDDKFYQKLRGQFPDAVFWQEIGEIFRQLQKQAAEIYNQSLVELYYEIFIKGKGFANASSAEHYLSDVCYTRAAELFKNAAIASGLRGKVKSNFRLKELKNMKSGLPTTKSDNFPIPLVKQKGGKYTGFEISSHNDDFIIKIPFGRWQVKKEIDKYRPWEKFDFEQVRKSPKPISLLLSTQRRKRNKGWSKDEGTEAEIRRVMNGDYQTSYIEVKRGSKIGEKSAWMLNLSIDVPKIDKGVDPSIIGGIDVGVKSPLVCAINNALSRYSISDNDLFHFNKKMFARRRILLKKNRHKRAGHGAKNKLRPISILTEKSKRFRKKLIERWACEIADFFVKNKVGTVQMENLESMKRKEDSYFNIRLRGFWPYAEMQNKIKFKLKQYGIEIRKVAPNNTSKTCSKCGHLNNYFNFEYRRKNKFPHFKCEKCNFKENADYNAALNISNPKLKSTKEEP

SEQ ID NO: 1715 - protein, 726 aa, synthetic construct
SEVEFSHEYWMRHALMLAKRARDEREVPVGAVLVLNNRVIGEGWNRAIGLHDPTAHAEIMALRQGGLAMQNYRLVDATLYVTFEPCVLCAGAMVHSRIGRVVFGVRNSKRGAAGSLMNVLNHPGMNHRVEITGGILADECAALLCDFYRMPRQVFNAQKKARSNINSGGSSGGSSGSETLGTSESATPKSSGGSSGGSAKNTITKALKLRIVRPYNSAEVEKIVADEKNNRERIALEKNKDKVKEACSKHLKVAAYCTTQVERNACLFCKARKLDDKFYQKLRGQFPDAVFWQEIGEIFRQLQKQAAEIYNQSLIELYYEILIKGKGFANASSVEHYLSDVCYTRAAELFKNAAIASGLRGKVKSNFRLKELKNMRSGLPTTKSDNFPIPLVKQKGGQYAGFEISSHNDDFIIKIPFGRWQVKEEIDKYRPWEKFDFEQVRKSPKPISLLLSTQRRKKNKGWSKDEGTEAEIRRVMNGDYQTSYIEVKRGSKIGEKSAWMLNLSIDVPKIDKGVDPSIIGGIDVGVKSPLVCAINNSSSRYSICDNDLFRFNKKMFARRRILLKKNRHKRAGHGAKNKLKPITILTKKSERFRKKLIERWVCEVADFFIKNKVGTVQMENLESMKRREDSYFNTRLRGFWPYAEMQNKIEFKLKQYGIEIRKVAPNNTSKTCSKCGHLNNYFNFEYRKKSKFPHFKCEKCNFREDADYNAALNISNPKLKSTKEEP

SEQ ID NO: 1716 - protein, 726 aa, synthetic construct; identical to SEQ ID NO: 1553

SEQ ID NO: 1717 - protein, 726 aa, synthetic construct
SEVEFSHEYWMRHALSLAKRARDEREVPVGAVLVLNNRIIGEGWNRAIGQHDPTAHAEIMALRQGGLVMQNYRLTDATLYVTFEPCVMCAGAMVHSRIGRVVFGVRNSKRGAAGSLMNVLNYPGVNHCVEITEGILVDECAALLCDFYRMPRQVLNAQKKAQSSISSGGSSGGCSGSEMPGASESVTPKSSGGSSAGSTKNTITKTLKLRIVRPYNSAEVEKIVADEKNSREKIALERNKDNVKEACSEHLKVAAYCTTQVERNACLFCKARKLDDRFYQKLRGQFPDAVFWQEAGEIFRQLQRQAAEIYNQSLIELYYEIFIKGKGFANASSVEHYLSDVCYTRAAELFKNAAIASGLRGKVKSNFRLKELKNMKSGLPTTKSDNFPIPLVKQKGGQYTGFEISSHNDDFIIKIPFGRWQMKKEIDRYRPWEKFDFEQVRKSPKPISLLLSTQRRKRNKGWSKDEGTEAEIRRVMNGDYQTSYIEVKRGSKIGEKSAWMLSLSIDVPKIDKGVDPSIIGGIDVGVKSPLVCAINNAFCRYSISDNDLFHFNKKMFARRRILLKKSRHKRAGHGAKNKLKPISILTEKSKRFRKKLIERWACEIADFFIKNKVGTVQMENLESMKRKEDSYFNIRLRGFWPYAEMQNKIEFKLKQYGIEIRKVAPNNTSKTCSKCGHLNNYFNFEFRKKNKFPHFKCEKCNFKEDADYNAALNISNPKLKSTKEEP

SEQ ID NO: 1718 - protein, 726 aa, synthetic construct
SEAEFSHEYWMRHALTLAKRARDEREVPVGAVLVLNNRVIGEGWNRAIGLHDPTAHAEIMALRQGGLVMQNYRLTDATLYVTFEPCVMCAGAMIHSRIGRVVFGVRNSKRGAAGSLMNVLNYPGMNHCVEITEGILVDECAALLCDFYRMPRQVLNAQKKAQSGISSGGSSGGSCCSETPGASESVTPKSSGGSSAGSTKNTITKTLKLRIVRPYNSAEVEKIVADEKNSREKIALEKNKDKVKEACSKHLKVAAYCTTQVERNACLFCKARKLDDRFYQKLRGQFPDAVFWQETGEIFRQLQRQAAEIYNQSLIELYYEILIKGKGFANASSVEHYLSDVCYTRAAELFKNAAIASGLRGKVKSNFRLKELKSMKSGLPTTKSDNFPIPLVKQKGGQYTGFEISSHNDDFIIKIPFGRWQVKEEIDKYRPWEKFDFEQVRKNPKPISLLLSTQRRKGNKGWSKDEGTEAEIRKVMNGDYQTSYIEVKRGSKIGEKSAWMLNLSIDVPKIDKGVDPSIIGGIDVGVKSPLVCAINNAFSRYSISDNDLFRFNKKVFARRRILLKKNRHKRAGHGTKNKLKPITILTEKSKRFRKKLIERWACEIADFFIKNKVGTVQMENLESMKRKEDSYFNIRLRGFWPYAEMQNKIEFKLKQYGIKIRKVAPNNTSRTCSKCGHLNNYFSFEYRKKNKFPHFKCEKCNFKEDADYNAALNICNPKLKSTKEEP

SEQ ID NO: 1719 - protein, 726 aa, synthetic construct
SEVEFSHEYWMRHALTLAKRARDEREVPVGAVLVLNNRVIGEGWNRAIGLHDPTAHAEIMALRQGGLVMQNYRLTDATLYVTFEPCVMCAGAMVHSRIGRVVFGVRNSKRGAAGSLMNVLNYPGMNHRVEITEGILADECAALLCDFYRMPRQVFGARRKAQSSINPGGSSGGSSGSETPGTSESPTPESPGGSSGGSAKNTITKTLKLRIVRPYNSPEVEKIVADEKNNREKIALEKNKDKVKEACSKHLKVASYCTTQVERNACLFCKARKLDDKFYQKLRGQFPDAVFWQELGGIFRQLQKQAAEIYNQSLIELYYEIFIKGKGITNASRVEHYLSDVCYTRAAELFKNAAIASGLRSKVRSNFRLKELKNMKSGLPTTKSDNFPIPLVKQKGGQYTGFEISSHNDDFIIKIPFGRWQVKKEIDKYRPWEKFDFEQVRKSPKPISLLLSTQRRKRNKGWSKDEGTEAEIRKVMNGDYQTSYIEVKRGSKIGEKSAWMLSLSIDVPKIDRGVDPSIIGGIDVGVKSPLVCAINNAFCRYSISDNDLFHFNKKMFARRRILLKKSRHKRAGHGAKNKLKPISILTEKSKRFRKKLIERWACEIADFFIKNKVGTVQIENLESMKRKEDSYFNIRLRGFWPYAEMQNKIEFKLKQYGIEIRKVAPNNTSKTCSKCGHLNSYFNFEYRKKNKFPHFKCEKCSFRENADYNAALNISNPKLRSTKEEP

SEQ ID NO: 1720 - protein, 726 aa, synthetic construct; identical to SEQ ID NO: 684

SEQ ID NO: 1721 - protein, 726 aa, synthetic construct
SEVEFSHEYWMRHALTLAKRARDEREVPVGAVLVLNNRVIGEGWNRAIGLHDPTAHAEIMALRQGGLVMQNYRLTDATLYVTFEPCVMCAGAMIHSRIGRVVFGVRNSKHGAAGSLMNVLNYPGMNHRVEITEGILADECAALLCDFYRMPRQVFNARKKTQSSINPGGPSGGSSGSETPDTSESATPESSGGSFGGSAKNTITKTLQLRIVRPYNSAEVEKIVADEKNSREKIALEKNKDKVKEACGKHLKVASYCTTQVERNACLFCKARKLDDKFYQKLRGQFPDAVFWQELGEIFRQLQKQAAEIYNQSLIELYYEIFIKGKGFANASSVEHYLSDVCYTRAAELFKNAAIASGLRGKVKSNFRLKELKNMKSGLPTTKSDNFPIPLVKQKGGQYTGFEISSHNDDFIIKIPFGRWQVKKEIDKYRPWEKFDFEQVRKSPKPISLLLSTQRRKRSKGWSKDEGTEAEIRKVMNGDYQTSYIEVKRGSKVGEKSAWMLNLSIDVPKVDKGVDPSIIGGIDVGVKSPLVCAINNALSRYSISDNDLFRFNKKMFARRRILLKKNRHKRAGHGAKNKLKPISILTEKSGRFRKKLIERWACEIADFFIKNKVGTVQMENLESMKRKEDSYFNIRLRGFWPYAEMQNKIEFKLKQYGIEIRKVAPDNTSKTCSKCGHLNSYFNFEYRKKNKFPHFKCEKCNFKEDADYNAALNISNPKLKSTKEEP

SEQ ID NO: 1722 - protein, 726 aa, synthetic construct
SEVEFSHEYWMRHALTLAKRARDEREVPVGAVLVLNNRVIGEGWNRAIGLYDPTAHAEIMALRQGGLVMQNYRLTDATLYVTFEPCVMCAGAMIHSRIGRVVFGVRNSKRGAAGSLMNVLNYPGVNHCVEITEGILVDECAALLCDFYRMPRQVFNARKKARSNINSGGSSGGSRGSETPGTSGSTTPEGSGSSSGGSVKNTITKTLKLRIVRPYNSAEVEKIVADEKNNREKIALEKNKDKVREACSKHLKVAAYCTTQVERNACLFCKARRLDDKFYQKLRGQFPDAVFWQEIGEIFRQLQKQAAEIYNQSLVELYYEIFIKGKGIANASSVEHYLSDVCYTRAAELFKNAAIASGLRGKVKSNFRLKELKNMRSGLPTTKSDNFPIPLVKQKGGQYAGFEICSHNDDFIIKIPFGRWQVKKEIDKYRPWEKFDFEQVRKSPKPISLLLSTQRRKRNKGWSKDEGTEAEIRKVMNGDYQTSYIEVKRGSKIGEKSAWMLNLSIDVPKIDKGVDPSIIGGIDVGVKSPLVCAINSAFSRYSISDNDLFHFNKKMFARRRILLKKNRHKRAGHGAKNKLKPISILTEKSKRFRKKLIERWACEIADFFIKNKVGTVQMENLESMKRKEDSYFNIRLRGFWPYAEMQNKIEFKLKQYGIEIRKVAPNNTSKTCSKCGHLNNNFNFEYRRKNKFPHFKCEKCNFKEDADYNAALNISNPKLKSTKEEP

SEQ ID NO: 1723 - protein, 726 aa, synthetic construct
SEVEFSHEYWMRHALTLAKRARDEREVPVGAILVLNNRVIGEGWNRAIGLHDPTAHAEIMALRQGGLVMQNYRLIDATLYVTFEPCVMCAGAMIHSRIGRVVFGVRNSKHGAAGSLMNVLNYPGMNHRVEITEGILADECAALLCDFYRMPRQVFNARKKAQSSINPGGPSGGSSGSETPDTSESAAPESSGGNSGGSAKNTITKTLKLRIVRPYNSAEVEKIVADEKNNREKVALEKNKDKVKEACSKHLKVAAYCTTQVERNACLFCKARRLDDKFYQKLRDQFPDAVFWQEIGEIFRQLQKQAAEIYNQSLVELYYEIFIKGKGIANASSVEHYLSDVCYTRAAELFKNAAIASGLRNKIKSNFRLKELRNMKSGLPTTKSDNFPIPLVRQKGGQYTGFEISNHNGDFIIKVPFGRWQVKKEICKHRPWEKFDFEQVRKSPKPISLLLSTQRRKRNKGWSKDEGTEAEIRKVMNGDYQTSYIEVKRGSKIGEKSAWMLNLSIDVPKIDKGVDPSIIGGIDVGVKSPLVCAINNALSRYSISDNDLFHFNKKMFARRRILLRKNRHKRAGHGARNKLKPVTVLTEKSERFRKKLIERWACEIANFFIKNKVGTVQMENLESMKRREDSYFNIRLRGFWPYAEMQSKIEFKLKQYGIKIRKVAPNNTSKTCGKCGHLNNYFNFEFRKKNKFPHFKCEKCNFKEDADYNAALNISNPKLKGTKEEP

SEQ ID NO: 1724 - protein, 726 aa, synthetic construct
NEVEFSHEYWMRRALTLAKRARDEREVPVGAVLVLNNRVIGVGWNRAVGLHDPTAHAEIMALRQGGLVMQNYRLIEATLYVTFEPCIMCAGAMIHSRIGRVVFGVRNSKRGAAGSLMNVLNYPGMNHRVEITEGILADECAALLCDYYRMPRQVFNARKKAQSSINSGGSSDGGSDSETPGTSESATPESSGGSSGGSAKNTITKTLKLRIVRPYNSAEVEKIVADEKNNREKIALEKNKDKVKEACSEHLKVAAYCTTQVERSACLFCKARKLDDKFYQKLRGQFPDAVFWQEIGEILRQLQKQAAEIYNQSLIELYYEIFIKGRGFANASSVEHYLSDVCYTRAAELFKNAAIASGLRGKVKSSFRLKELKNMKSGLPTTKSDNFPIPLVKQKGGQYTGFEISSHNDDFIIKIPFGRWQVKKEIDKYRPWEKFDFEQVRKSPKPISLLLSTQRRKRNKGWGKDEGTEAEIRKVMNGDYQTSYIEVKRGSKIGEKSAWMLNLSIDVPKIDKGVDPSIIGGIDVGVKSPLVCAINNAFSRYSISDNDLFRFNKKMFARRRILLKKSKHKRAGHGAKNKLKPITILTEKSGRFRKKLIERWACEIADFFIKNKVGTVQMENLESMKRREDSYFNIRLRGFWPYAEMQSKIEFKLKQYGIKIRKVAPNNTSKTCSKCGHLNNYFNFEFRKKNKFPHFKCEKCNFKEDADYNAALNISNPKLKSTKEEP

SEQ ID NO: 1725 - protein, 726 aa, synthetic construct
SEVEFSHEYWMRHALTLAKRARDEREVPVGAVLVLNNRVIGEGWNRAIGLHDPTAHAEIMALRQGGLVMQNYRLTDATLYVTFEPCVMCAGAMIHSRIGRVVFGVRNSKRGAAGSLMNVLNYPGMNHCVEITEGILVDECAALLCDFYRMPRQVLNAQKKAQSSISSGGSSDGSSGSETPGTSESATPESSGGGSSGSARNTITKTLQLRIVRPYNSAEVEKIVADEKNNREKIALEKNKGKVREACNKHLKVASYCTTQVERNACPFCKARKLDDKFYQKLRGQFPDAVFWQELGEILRQLQKQAAEIYNQSLIELYYEIFIKGRGFANASSVEHYLSDVCYTRAAELFKNAAIASGLRGKVKSNFRLKELRSMKSGLPTTKSDNFPIPLVKQKGGQYTGFEISNHNSDFIIKIPFGRWQAKKEIDKYRPWEKFDFEQVRKSPKPISLLLSTQRRKRNKGWSKDEGTEAEIRKVMNGDYQTSYIEVKRGSKIGEKSAWMLNLSIDVPKIDKGVDPSIIGGIDVGVKSPLVCAINNAFSRYSISDNDLFHFNKKMFARRRILLKKNRHKRAGHGATNKLKPITILTEKSGRFRKKLIERWACEIADFFIKNKVGTVQMENLESMKRREDSYFNIRLRGFWPYAEMQNKIEFKLKQYGIEIRKVAPNNTSKTCSKCGHLNNYFNFEYRKKNKFPHFKCEKCNFKENADYNAALNISNPKLKSTKEEP

SEQ ID NO: 1726 - protein, 726 aa, synthetic construct
SEVEFSHEYWMRHALTLARRARDEREVPVGAILVLNNRVIGEGWNRAIGLHDPTAHAEIMALRQGGLVMQNYRLVDATLYVTFEPCVMCAGAMIHSRIGRVVFGVRNNKHGAAGSLMNILNYPGMNHRVEITEGILADECAALLCDFYRMPRQVFNAQKKARSNINSGGSSGGSSGSETPGTSESPTPESSGGGSAGSTKNTITKTLKLRIVRPYNSAEVEKIVADEKNNREKIALEKNRDKVKEACSKHLKVAAYCTTQVERNACLFCKARKLDDKFYQKLRGQFPDAVFWQELGGILRQLQKQAAEIYNQSLIELYYEIFIKGRGFANASSVEHYLSDVCYTRAAELFKNAAIASGLRGKVKSNFRLKELRNMKSGLPTTKSDNFPIPLVRQKGGQYTGFEISNYNGDFIIKIPFGRWQVKKEINKHRPWEKFDFEQVRKSPKPISLLLSTQRRKRNKGWSKDEGTEAEIRKAMNGDYQTSYIEVKRGSKIGEKSAWMLSLSIDVPKIDKGVDPRIIGGIDVGVKSPLVCAINNVLSRYSISDNDLFHFNKKMFARRRILLKKNGHKRAGHGAKNKLKPITIMTEKSKRFRKKLIERWACEIADFFIKNKVGTVQMENLESMKRKEDSYFNIRLRGFWPYAEMQNKIEFKLRQYGIVVRKVAPNNTSKTCSQCGHLNNYFNFEYRKKNKFPYFKCEKCNFKENADYNAALNISNPQLKSTKGEP

SEQ ID NO: 1727 - protein, 726 aa, synthetic construct
SEVEFSHEYWMRHALTLAKRARDEREVPVGAILVLNNRVIGEGWNRTIGLHDPTAHAEIMALRQGGLVMQNYRLTDATLYVTFEPCVMCAGAMIHGRIGRVVFGVRNSKRGAAGSLMNVLNYPGMNHCVEITEGILVDECAALLCDFYRMPRQVLNAQKKAQSSISSGGSSGGSSGGETPGASGSVTPKSSGGSSAGSTKDTITKTLKLRIVRPYNSAEVEKIVADEKNNREKIALEKNKDKVKEACSEHLKVAAYCTTQVERNACLFCKARRLDDKFYQKLRGQFPDAVFWQEIGEIFRQLQKQAAEIYNQSLVELYYEIFIKGRGFANASSVEHYLSGVCYTRAAELFKNAAIASGLRGKVKSNFRLKELKNMKSGLPTTKSDNFPIPLVKQKGGQYTGFEISSHNDDFIIKIPFGRWQVKKEIDKYRPWEKFDFEQVRKSPKPISLLLSTRRRKRNKGWSKDEGTEAEIKKVMNGDYQTSYIEVKRGSKIGEKSAWMLNLSIDVPKIDKGVDPSIIGGIDVGVKSPLVCAINNAFSRYSISDNDLFRFNKKMFARRRILLKKSRHKRAGHGAKNKLKPITILTEKSGRFRKKLIERWACEIADFFIKNKVGTVQMENLESMRRKEDSYFNIRLRGFWPYAEMQNKIEFKLKQYGIVVRKVAPNNTSKTCSKCGHLNNYFNFEYRRKNKFPHFKCEKCNFKENADYNAALNISNPKLKSTKEEP

SEQ ID NO: 1728 - protein, 726 aa, synthetic construct
SEVEFSHEYWMRHALTLAKRARDEREVPVGAVLVLNNRVIGEGWNRAIGLHDPTAHAEIMALRQGGLVMQNYRLTDATLYVTFEPCVMCAGAMIHSRIGRVVFGVRNSKRGAAGSLMNVLNYPGMNHRVEITEGILVDECAALLCDFYRMPCQVLNAQKKAQSTINSGGSSGGSSSSETPGTSGSATPEGSGGSSGGPAKNTITKTLKLRIVRPHNSAEVEKIVADEKNNREKIALEKNKDKVKEACSKHLKVASYCTTQVERNACMFCKARKLDDEFYQKLRGQFPDAVFWQELGEIFRQLQKQAAEIYNQSLIELYYEIFIKGKGFANASSVEHYLSDVCYTRAAELFKNAAIASGLRGKVKSNFRLKELKNMKSGLPTTKSDNFPIPLVKQKGGQYTGFEISSHNDDFIIKIPFGRWHVKKEIDKYRPWEKFDFEQVRKSPKPISLLLSTQRRKRNKGWGKDEGTEAEIRKVMNGDYQTSYIEVKRGSKIGEKSAWMLNLSIDVPKIDKGVDPSIIGGIDVGVKSPLVCAINNAFSRYSISDNDLFRFNKKMFARRRILLKKSKHKRAGHGAKNKLKPITILTEKSGRFRKKLIERWACEIADFFIKNKVGTVQMENLESMKRKEDSYFNIRLRGFWPYAEMQNKIEFKLKQYGIEIRKVAPNNTSKTCSKCGHLNNYFNFEYRRKNKFPHFKCEKCNFKENADYNAALNISNPKLKSTKEEP

SEQ ID NO: 1729 - protein, 726 aa, synthetic construct
SEVEFSHEYWMRHALTLAKRARDEREVPVGAILVLNNRVIGEGWNRAIGLHDPTAHAEIMALRQGGLVMQNYRLIDATLYVTFEPCVMCAGAMIHSRIGRVVFGVRNSKHGAAGSLVNVLNYPGMNHRVEITEGILADECAALLCDFYRMPRQVFNARKKAQSSINPSGSSDGGSGSETPGTSESATPESSGGSSSGSAKNTITKTLKLRIVRPYNSAEVEKIVADEKNNREKIALEKNKNKVKEACSEHLKVAAYCTTQVERSACLFCKARKLDDKFYQKLRGQFPDAVFWQETGEIFRQLQKQAAEIYNQSLIELYYEIFIKGKGFANASSVEHYLSDVCYTRAAELFKNAAIASGLRGKVKSNFRLKELKNMKSGLPTTKSDNFPIPLVKQKGGQYTGFEISSHNDDFIIKIPFGRWQVKKEIDKYRPWEKFDFEQVRKSPKPISLLLSTRRRKRNKGWSKDEGTEAEIRRVMNGDYQTSYIEVKRGSKIGEKSAWMLNLSIDVPKIDKGVDPSIIGGIDVGVKSPLVCAINNAFSRYSISDNDLFRFNKKMFARRRVLLKKNRHKRAGHGAKNKLKPISILTGKSERFRKKLIERWACEIADFFIKNKVGTVQMENLESMKRKEDSYFNTRLRGIWPYAEMQNKIEFKLKQYGIEIRKVAPNNTSKTCSKCGHLNNYFNFEYRKKNKFPHFKCEKCNFKEDADYNAALNISNPRLKGTKEEP

SEQ ID NO: 1730 - protein, 726 aa, synthetic construct
SEVEFSHEYWMRHALTLARRARDEREVPVGAVLVLNSRVIGVGWNRAVSLHDPTAHAEIMALRQGGLVMQNHRLIDATLYVTFEPCVMCAGAMVHSRIGRVVFGVRNSKRGAAGSLMNVLNYPGMNHRVEITEGILADECAALLCDFYRMPRQVFNAQRKAQSSINFGGSSGGSSGSVTPGTSESATPESSGGGFGGSAKNTITKTLQLRIVRPYNSAEVEKIVADEKSNREKIALEKNKDKVKEACSKHLKVASYCTTQVERNACLFCKARKLDDKFYQKLRGQFPDAVFWQEIGEIFRQLQKQAAEIYNQSLIELYYVIFIKGKGLVNASSVEHYLSDVCYTRAAELFKNAAIASGLRGKVKSNFRLKELKNMKSGLPTTKSDNFPIPLVKQKGGQYTGFEISSHNSDFIIKIPFGRWRVKKEIDKFRPWEKFDFEQVRKSPKPISLLLSTQRRKRNRGWSKDEGTEAEIRKVMNGDYQTSYIEVKRGSKIGEKSAWMLNLSIDVPKIDKGVDPSIIGGIDVGVKSPLVCAINNSFSRYSISDNDLFRFNKKVFARRRILLKKNRHKRAGHGTKNKLKPITILTEKSGRFRKKLIERWACEIADFFIKNKVGTVQMENLESMKRREDSYFNIRLRGFWPYAEMQNKIEFKLKQYGIKIRKVAPNNTSKTCSKCGHLNNYFSFEYRKKNKFPHFKCEKCNFKEDADYNAALNISNPKLKSTKEEP

SEQ ID NO: 1731 - protein, 726 aa, synthetic construct
SEVEFSHEYWMRHALTLAKRARDEREVPVGAILVLNNRVIGEGWNRAIGLHDPTAHAEIMALRQGGLVMQNYRLIDATLYVTFEPCVMCAGAMIHSRIGRVVFGVRNSKHGAAGSLMNVLNYPGMNHCVEITEGILVDECAALLCDFYRMPRQVLNAQKKAQSSISSGGSSGGSSGSETPGASGSVIPKSSGGSSAGSTKDTITKTLKLRIVRPYNSAEVEKVVADEKNNREKIAMEKNKDKVKEACSKHLKVASYCTTQVERNACLFCKARKLDDKFYQKLRGQFPDAVFWQELGGIFRQLQKQAAEIYNQSLVELYYEIFIKSKGIANASSVEHYLSNVCYTRAAELFKNAAIASGLRNKIKSNFRLKELRNMKSGLPTTKSDNFPIPLVKQKGGQYTGFEISSHNDDFIIKIPFGRWQVKKEIDKYRPWEKFDFAQVRKSPKPISLLLSTQRRKRNKGWSNDEGTEAEIRKVMNGDYQTSYIEVKRGSKIGEKSAWMLSLSIDVPKIDKGVDPSIVGGIDVGVKSPLVCAINNALGRFSISDNDLFHFNKKMFARRRILLRKNRHKRAGHGAKNKLKPISILTEKSRRFRKKLIERWACEIADFFIKNKVGTVQMEDLESMKRRGDSYFNIRLRGLWPYAEMQNKIEFKLKQYGIEIRKVAPNNTSKTCSKCGHLNNYFNFEYRKKNKFPHFKCEKCNFKENADYNAALNISNPKLKNTKEEP

SEQ ID NO: 1732 - protein, 726 aa, synthetic construct
SEVEFSHEYWMRHALTLAKRARDEREVPVGAILVLNNRVIGEGWNRAIGLHDPTAHAEIMALRQGGLVMQNYRLIDATLYVTFEPCVMCAGAMVHSRIGRVVFGVRNSKRGAAGSLMNVLDYPGMGHRVEITEGILADECAALLCDFYCMPRQVFNAQKRAQSSINPGGSSGGSSGSDTPGTSESATPESSGGGSSGSAKNTITKTLQLRIVRPYNSAEVEKIVADEKNNREKIALEKNKDKVREACSKHLKVASYCTTQVERNACPFCKARKLDDKFYQKLRGQFPDAVFWQELGEILRQLQKQAAEIYNQSLIELYYEIFIKGRGFANASSVEHYLSDVCYTRAAELFKNAAIASGLRGKVKGNFRLKELKNMKSGLPTTKSDNFPIPLVKQKGGQYTGFEISSHNDDFIIKIPFGRWQVKKEIDKYRPWEKFNFEQVRKSPKPISLLLSTQRRKRNKGWSKDEGTEAEIRKVMNGDYQTSYIEVKRGSKTGEKSAWMLNLSIDVPKIDKGVDPSIIGGIDVGVKSPLVCAINNAFSRYSISDNDLFRFNKKMFARRRILLMKNRHKRAGHGAKNKLKPISILTGKSERFRKKLIERWACEIADFFIKNKVGTVQMENLESMKRKEDSYFNIRLRGFWPYAEMQNKIEFKLKQYGIEIRKVAPNNTSKTCSKCGHLNNYFNFEYRKKNKFPHFKCEKCNFKENADYNAALNISNPKLKSTKGEP

SEQ ID NO: 1733 - protein, 726 aa, synthetic construct
SEVEFSHEYWMRHALTLAKRARDEREVPVGAVLVLNNRAIGEGWNRAIGLHDPTAHAEIMALRQGGLVMQNYRLTDATLYVTFEPCVMCAGAMIHSRIGRVVFGVRNSKRGAAGSLMNVLNYPGMNHCVEITEGILVDECAALLCDFYRMPRQVLSAQKKAQSSVSSGDSSGGSSGSETPGASGSVTPKSSVGSSAGSTKNTITKTLKLRIVRPYNSAEVEKIVADEKNNREKIALEKNRDKVKEACSKHLKVAAYCTTQVERNACLFCKARKLDDKFYQKLRGQFPDAVFWQELGGIFRQLQKQAAEIYNQSLIELYYEIFIKGKGITNAGRVEHYLSDVCYTRAAELFKNAAIASGLRSKVRSNFRLKELKSMKSGLPTTKSDNFPIPLVKQKGGQYTGFEISSHNSDFIIKIPFGRWQVKEEIDKYRPWEKFDFEQVRKSPKPISLLLSTQRRKKNKGWSKDEGTEAEIRRVMNGDYQTSYIEVKRGSKIGEKSAWMLNLSIDVPKIDKGVDPSIIGGIDVGVKSPLVCAISNAFSRYSISDNDLFHFNKKMFARRRILLKKSKHKRAGHGARNKLKPITVLTEKSERFRKKLIERWACEIANFFIKNKVGTVQMENLESMRRKEDSYFNIRLRGFWPYAEMQNKIEFKLKQYGIEIRKVAPNNTSKTCSMCGHLNNYFNFEYRKKNKFPHFKCEKCNFKENADYNAALNISNPKLKSTKEEP

SEQ ID NO: 1734 - protein, 726 aa, synthetic construct
SEVEFSHEYWMRHALTLAKRARDGREVPVGAVLVLNNRVIGEGWNRAIGLHDPTAHAEIMALRQGGLAMQNYRLTDATLYVTFEPCVMCAGAMIHSRIGRVVFGVRNSKRGAAGSLMNVLNYPGMNHCVEITEGILVDECAALLCDFYRMPRQVFNARKKAQSSIDSAGSPGGSSGSETPGDSESATSESSGGSSGGSAKNTITKTLKLRIVRPYNSAEVEKIVADEKNNREKIALEKNKDKVKEACSKHLKVASYCTTQVERNACLFCKARKLDDKFYQKLRGQFPDAVFWQELGEIFRQLQKQAAEIYNQSLIELYYEIFIKGKGIANASSVEHYLSDVCYTRAAELFKNAAIASGLRNKVKSNFRLKELRSMKSGLPTTKSDNFPIPLVRQKGGPYTGFEISNHNSDFIIKIPFGRWQAKKEIDKYRPWVKFDFEQVRKSPKPISLLLSTQRRKRNRGWSKDESTEAEIKKVMNGDYQTSYIEVKRGSKVGEKSAWMLNLSIDVPKIDKGVDPSIIGGIDVGVKSPLVCAINNAFSRYSISDNDLFRFNKKVFARRRILLKRNGHKRAGHGTKNKLKPITILTEKSERFRKKLIEKWACEIADFFIKNKVGTVQMENLESMKRKEDSYFNIRLRGFWPYAEMQNKIEFKLKQYGIEIRKVAPNNTSKTCSKCGHLNNYFNFEYRKKNKFPHFKCEKCNFKENADYNAALNISNPKLKSTKEEP

SEQ ID NO: 1735 - protein, 726 aa, synthetic construct
GEDEFSHEYWMRHALTLAKRARDGREVPVGAVLVLNNRVIGEGWNRAIGLHDPTAHAEIMALRQGGLVMQNYRLIDATLYVTFEPCVMCAGAMVHSRIGRVVFGVRNSKRGAAGSLMNVLDYPGMGHRVEITEGILADECAALLCDYYRMPRQVFNARKKAQSSINSSGSSDGGSGSETPGTSESATPESSGGSSGGSAKNTITKTLKLRIVRPYNSAEVEKIVAVEKNNREKIALEKNKDKVKEACSEHLKVAAYCTTQVERSACLFCKARKLDDKFYQKLRGQFPDAVFWQELGEVLRQLQKQAAEIYNQSLIELYYEIFIKGKGFANASSVEHYLSDVCYTRAAELFKNAAIASGLRGKVKSNFRLKELKNMKSGLPTTKSDNFPIPLVKQKGGQYTGFEISSHNNDFIIKIPFGRWQVKEEIDKYRPWEKFDFEQVRKSPKPISLLLSTQRRKRNKGWSKDEGTEAEIRKVMNGDYQTSYIEVKRGSKIGEKSAWMLNLSIDVPKIDKGVDPSIIGGIDVGVKSPLVCAINNAFIRYSISDNDLFHFNKKMFARRRILLKKNRHKRAGHGAKNKLKPISILTEKSKRFRKKLIERWACEIADFFIKNKVGTVQMENLESMKRKEDSYFNIRLRGFWPYAEMQNKIEFKLKQYGIEIRKVAPNNTSKTCAKCGHLNNYFNFEFRKKNKFPHFKCEKCNFKENADYNAALNISNPKLKSTKEEP

SEQ ID NO: 1736 - protein, 726 aa, synthetic construct
SEVEFSHEYWMRHALTLAKRARDKHEVPVGAVLVLDNRVIGEGWNRATGQNDPTAHAEIMALRQGGLVMQNHRLIDATLYVTFEPCVMCAGAMIHSRIGRVVIGVRNSKRGAAGSLMNVLNHPGMNHRVEITEGILADECAALLCDFYRMPRQVLNAQEKAQSSINSGGSSGGSSGSETPGTSESATPGSSGGSSGGSAKNTITKTLKLRIVRPYNSAEVEKIVADEKNSREKIALEKNKDKVKEACGKHLKVAAYCTTQVERNACLFCKARKLDDKFYQKLRGQFPDAVFWQEIGEIFRQLQKQAAEIYNQSLIELYYEIFIKGKGFANASSVEHYLSDVCYTRAAELFKNAAIASGLRGKVKSNFRLKELKNMRSGLPTTKSDNFPIPLVKQKGGQYAGFEISSHNDDFIIKIPFGRWQVKKEIDKYRPWEKFDFEQVRKSPKPISLLLSTRRRKRNKGWSKDEGTEAEIRKVMNGDYQTSYIEVKRGSKIGEKSAWMLNLSIDVPKIDKGVDPSIIGGIDVGVKSPLVCAINNAFGRYSISDNGLFHFNKKMFARRRVLLKKNRHKRAGHGAKNKLKPITILTEKSKRFRKKLIERWACEIADFFIKNKVGTVQMENLESMKRKEDSYFNIRLRGFWPYAEMQDKIEFKLKQYGIEIRKVAPNNTSKTCSRCGHLNNYFNFEYRKKNKFPHFKCEKCNFREDADYNAALNISNPKLKSTKEEP

SEQ ID NO: 1737 - protein, 726 aa, synthetic construct
SEVEFSHEYWMRHALTLAKRARDEREVPVGAVLVLNNRVIGEGWNRAIGLHDPTAHAEIMALRQGGLVMQNYRLIDATLYVTFEPCVMCAGAMIHSRIGRVVFGVRNNKHGAAGSLVNVLDYPGMNHRVEITEGILADECAALLCDFYRMPRQVFNARKKAQSSISPGGSSGGSSGSETPGTSESATPESSGGSSGGSAKNTITKTLKLRIVRPYNSAEVEKIVADEKNSREKIALEKNKDKVKEACSKHLKVAAYCTTQVERNACLFCKARKLDDKFYQKLRGQFPDAVFWQEIGEVFRQLQKQAAEIYNQSLIELYYEIFIKGKGFANASSVEHYLSDVCYTRAAELFKNAAIASGLRGKVKSNFRLKELKNMKSGLPTTKSDNFPVPLVKQKGGQYTGFEISNHNGDFIIKIPFGRWQVKKEINKYRPWEKFDFEQVRKNPKPISLLLSTQRRKRNKGWSKDEGTEAEIRKVMNGDYQTSYIEVKRGSKIGEKSAWMLNLSIDVPKIDKGVNPSIIGGIDVGVKSPLVCAINNALSRYSISDNDLFHFNKKMFARRRILLKKNRHRRAGHGARNKLKPITVLTEKSERFRKKLIERWACEIANFFVKNRVGTVQMENLESMKRKEDSYFNIRLRGFWPYAEMQNKIEFKLKQYGIEIRKVAPNNTSKTCSKCGHLNNYFNFEYRKKNKFPHFKCEKCNFKENADYNAALNISNPMLKSTKEEP

SEQ ID NO: 1738 - protein, 726 aa, synthetic construct
SEVEFSHEYWMRHALTLAKRARDEREVPVGAVLVLNNRVIGEGWNCTIGLHDPTAHAEIMALRQGGLVMQNCRLTDATLYVTFEPCVMCAGAMIHSRIGRVVFGVRNSKRGAAGSLMNVLNYPGMNHCVEITEGILADECAALLCDFYRMPRQVFNARKKAQSSINPGGSSGGSSGSETPGTSESATPESSGGSSGSSAKNTITKTLKLRIVRPYNSAEVEKIVADEKNNREKIALEKNKDKVKEACSKHLKVAAYCTTQVERNACLFCKARRLDDKFYQKLRGQFPDAVFWQEIGEIFRQLQKQAAEVYNQSLVELYYEILIKGKGIANASSVEHYLSDVCYTRAAELFKNAAIASGLRNKIKSNFRLKELRNMKSGLPTTKSDNFPIPLVRQKGGQYTGFEISNHDGDFIIKIPFGRWQVKKEINKHRPWEKFDFEQVRKSPKPISLLLSTQRRKRNKGWSKDEGTEAEIRKVMNGDYQTSYIEVKRGSKIGEKSAWMLNLSIDVPKIDKGVDPSIIGGIDVGVKSPLVCAINNALSRYSISDNDLFHFNKKMFARRRILLRKNRHKRAGHGAKNKLKPITIMTERSKRFRKKLIERWACEIADFFIKNKVGTVQMENLESMKRREDSYFNIRLRGFWPYAEMQNKIEFKLKQYGIVVRKVAPNNTSKTCSKCGHLNNYFNFEYRKKNKFPHFKCEKCNFKEDADYNAALNISNPKLKSTKGEP

SEQ ID NO: 1739 - protein, 726 aa, synthetic construct
SEVEFSHEYWMRHALTLAKRARDEREVPVGAVLVLNNRVIGEGWNRAIGLHDPTAHAEIMALRQGGLVMQNYRLIDATLYVTFEPCVMCAGAMIHSRIGRVVFGVRNNKHGAAGSLVNVLNYPGMNHRVEITEGILADECAALLCDFYRMPRQVFNARKKAQSSINPGGSSGGSSGSETPGTSESATPESSGGSSGSSAKNTITKTLKLRIVRPYNSAEVEKIVADEKNNREKIALEKNKDKVKEACSKHLKVAAYCTTQVERNACLFCKARKLDDKFYQKLRGQFPDAVFWQEISEIFRQLQKQAAEIYNQSLIELYYEIFIKGKGITNASRVEHYLSDVCYTRAAELFKNAAIASGLRSKVRSNFRLKELKNMKSGLPTTKSDNFPIPLVKQKGGQYTGFEISSHNSDFIIKIPFGRWQEKEEIDKYRPWEKFDFEQVRKSPKPISLLLSTQRRKRNKGWSKDEGTEAEIRKVMNGDYQTSYIEVKRGSKIGEKSAWMLNLSIDVPKIDKGVDPSIIGGIDVGVKFPLVCAINNAFSRYSISDNDLFHFNKKMFARRRILLKKNRHKRAGHGAKNKLKPITILTEKSVRFRKKLIERWACEIADFFIKNKVGTVQMENLESMKGKEDSYFNIRLRGFWPYAEMQNKIEFKLKQYGIEIRKVAPNNTSKTCSKCGHLNNYFNFEYRKRNKFPHFKCERCNFKENADYNAALNISNPKLKSTKGEP

SEQ ID NO: 1740 - protein, 726 aa, synthetic construct
SEVEFSHEYWMRHALTLAKRARDEREVPVGAILVLNNRVIGEGWNRAIGLHDPTAHAEIMALRQGGLVMQNYRLIDATLYVTFEPCVMCAGAMIHSRIGRVVFGVRNSKHGAAGSLVNVLNYPGMNHRVEITEGILADECAALLCDFYRMPRQVFNARKKAQSSISPGGSSGGSSGSETPGASGGVTPKSSGGSSAGSTKDTITKTLKLRIVRPYNSAEVEKIVADEKNSREKIALEKNKDKVKEACSEHLKVAAYCTTQVERNACPFCKARKLDDKFYQKLRGQFPDAVFWQELGEILRQLQKQAAEIYNQSLIELYYEIFIKGKGIANASSVEHYLSDVCYTRAAELFKNAAIASGLRGKVKSNFRLKELRNMKSGLPTTKSDNFPIPLVRQKGGQYTGFEISSRNDDFIIKIPFGRWQVKKEINKHRPWEKFDFEQVRKSPKPISLLLSTQRRKRNKGWSKDEGTEAEIRKVMNGDYQTSYIEVKRGSKIGEKSAWMLNLSIDVPKIDKGVDPSIIGGIDVGVKSPLVCAINNALSRYSISDNDLFHFNKKMFARRRILLRKNRHKRAGHGAKNKLKPITMMTEKSKRFRKKLIERWACEIADFFVKNKVGTVQMENLESMKRKEDSYFNIRLRGLWPYAEMQNKIEFKLKQYGIEIRKVAPNNTSKTCSKCGHLNNYFNFEYRKKNKFPHFKCEKCNFKENADYNAALNISNPKLKSTKEEP

SEQ ID NO: 1741 - protein, 726 aa, synthetic construct
SEVELSHEYWMRHALTLAKRARDEREVPVGAVLVLNNRVIGEGWNRAIGLHDPTAHAEIMALRQGGLVMQNYRLTDATLYVTFEPCVMCAGAMIHSRIGRVVFGVRNSKRGAAGSLMNVLNYPGMNHCVEITEGILVDECAALLCDFYRMPHQVLNAQKKAQSSISPGGSSGGSSGSETPGASESVTPKSSGGSSGGSAKNTITKTLQLRIVRPYNSAEVEKIVADEKNNREKIALEKNKDKVKEACSKHLKVASYCTTQVERNACPFCKARKLDDKFYQKLRGQFPDAVFWQEVGVIFRQLQKQAAEIYNQSLIELYYEIFIKGKGIANASSVGHYLSDVCYTRAAGLFKNAAIASGLRGKIKSNFRLKELKNMKSGLPTTKSDNFPIPLVKQKGGQYTGFEISSHNDDFIIKIPFGRWQVKKEIDKYRPWEKFDFEQVRKSPKPISLLLSTQRRKKNKGWSKDEGTEAEIRRVMNGDYQTSYIEVKRGSKIGEKSAWMLNLSIDVPKIDKGVDPSIIGGIDVGVKSPLVCAINNAFSRYSISDNELFHFNKKMFARRRILLKKNRHKRAGHGAKNKLKPISILTEKSERFRKKLIEKWACEIADFFIKNKVGTVQMENLESMKRKEDSYFNIRLRGFWPYAEMQNKIEFKLKQYGIEIRKVAPNNTSKTCSKCGHLNNYFNFEYRKKNKFPHFKCEKCNFKENADYNAALNISNPKLKSTKEGP

SEQ ID NO: 1742 - protein, 726 aa, synthetic construct
SEDEFSHEYWMRHALTLAKRARDGREVPVGAVLVLNNRVIGEGWNRAIGLHDPTAHAEIMALRQGGLVMQNYRLIDATLYVTFEPCVMCAGAMVHSRIGRVVFGVRNSKRGAAGSLMNVLDYPGMGHRVEITEGILADECAALLCDFYCMPRQVFNAQKRAQSSINSGGSSGGSCGSDTPGTSESATPESSGGGSSGSAKNTITKTLQLRIVRPYNSAEVEKIVADEKNNREKIALEKNKDKVREACSKHLKVASYCTTQVERNACPFCKARKLDDKFYQKLRGQFPDAVFWQELGEILRQLQKQAAEIYNQSLIELYYEIFIKGRGFANAGSVEHYLSDVCYTRAAELFKNAAIASGLRGKVKSNFRLKELKNMKSGLPTTKSDNFPIPLVKQKGGQYTGFEISSHNDDFIIKIPFGRWQVKKEIDKYRPWEKFDFEQVRKSPKPISLLLSTQRRKRNRGWSKDEGTEAEVKKVMNGDYQISYIEVKRGSKIGEKSAWTLNLSIDVPKIDKGVDPSIIGGIDVGVKSPLVCAISNAFSRYSISDNDLFHFNKKMFARRRILLKKSKHKRAGHGVKNKLKPITILTEKSRRFRKKLIERWACEIADFFIKNKVGTVQMENLEGMKRKEDSYFNIRLRGFWPYAEMQNKIEFKLKQYGIEIRKVAPNNTSKTCSKCGHLNNYFNFEYRKKNKFPHFKCEKCSFKENADYNAALNISNPKLKSTKEEP

SEQ ID NO: 1743 - protein, 726 aa, synthetic construct
GEVEFSHEYWMRHALTLAKRARDEREVPVGAVLVLNNRVIGEGWNRAIGLHDPTAHAEIMALRQGGLVMQNYRLIDATLYVTFEPCVMCAGAMIHSRIGRVVFGVRNSKHGAAGSLVNVLNYPGMNHRVEITEGILMDECAALLCDFYRMPRQVLNAQKKAQSSINSGGSSGGSSGSETPGASESVTPKSSGGGSSGSAKNTITKTLQLRIVRPYNSTEVEKIVADEKNNREKIALEKNKDKVKEACSEHLKVAAYCTTQVERSACLFCKARKLDDKFYQKLRGQFPDAVFWQEIGEIFRQLQKQAAEIYNQSLIELYYEIFIKGKGFANASSVEHYLSDVCYTRAAELFKNAAIASGLRGKVKSNFRLKELKNMKSGLPTTKSDNFPIPLVKQKGGQYTGFEISSHNDDFIIKIPFGRWQVRKEIDKYRPWEKFDFEQVRKSPKPISLLLSTQRRKRNKGWSKDEGTEAEIRKVMNGDYQTSYIEVKRGSKTGEKSAWMLNLSIDVPKIDKGVDPSIIGGIDVGVKSPLVCAINNAFSRYSIGDNDLFHYNKKMFARRRILLKKNRHKRAGHGAKNKLKPISILTEKSKRFRKKLIERWACEIADFFIKNKVGTVQIENLESMKRKEDSYFNIRLRGFWPYAEMQNKIEFKLKQYGIEIRKVAPNNTSKTCSKCGHLNSYFNFEYRKKNKFPHFKCEKCNFKENADYNAALNISNPKLKSTKEEP

SEQ ID NO: 1744 - protein, 726 aa, synthetic construct
SEVGFSHEYWMRRALTLAKRARDEREVPVGAVLVLNNRVIGVGWNRAIGLHDPTAHAEIMALRQGGLVMQNYRLVDATLYVTFEPCVMCAGAMIHSRIGRVVFGVRNNKHGAAGSLMNVLNYPGMNHRVEITEGILADECAALLCDFYRMPRQVFNARKKAQSSINPGGSSGGSSGSETPGTSESATPESSGGSSGSSAKNTITKTLKLRIVRPYNSAEVEKIVADEKNNREKIALEKNKDKVKEACSKHLKVAAYCTTQVERNACLFCKARRLDDKFYQKLRGQFPDAVFWQELGEIFRQLQKQAAEVYNQSLIELYYEIFIKGKGFANASRMEHYLSDVCYTRAAGLFKNAAIASGLRGKIKSNFRLKELKSMKSGLPTTRSDNFPIPLVKQKGGQYTGFEISNHDSDFIIKIPFGRWQVKKEIDKYRPWEKFDFEQVRKSPKPISLLLSTQRRKGNRGWSKDEGTEAEIRKVMNGDYQTSYIEVKRGSKIGEKSAWMLNLSIDVPKIDKGVDPSIIGGIDVGVKSPLVCAINNAFSRYSISDNDLFRFNKKVFARRRILLKRNRHKRAGHGTKNKLKPITILTEKSGRFRKKLIERWACEIADFFVKNKVGTVQMENLESMKRKEDSYFNIRLRGFWPYAEMQNKIEFKLKQYGIEIRRVAPNNTSRTCSKCGHLNNYFNFEYRRKYKFPHFKCEKCNFKEDADYNAALNISNPKLKSTKEEP

SEQ ID NO: 1745 - protein, 726 aa, synthetic construct
SEIEFSHEYWMRHALTLARRARDEREVPVGAILVLNNRVIGEGWNRAIGLHDPTAHAEIMALRQGGLVMQNYRLIDATLYVTFEPCVMCAGAMIHSRIGHVVFGVRNNKHGAAGSLVNVLDYPGMNHRVEITEGILADECAALLCDFYRMPRQVFNARKKAQSSISPGGSSGGSSGSETPGTSESATPESSGGSSGGSAKNTITKTLKLRIVRPYNSAEVEKIVADEKNNREKIALEKNKDKVKEACSKHLKVAAYCTTQVERNACLFCKARKLDDKFYQKLRGQFPDAMFWQEIGEVFRQLQKQAAEIYNQSLIELYYEIFIKGKGFANASSVEHYLSDVCYTRAAELFKNAAIASGLRNKIKSNFRLKELRNMKSGLPTTKSDNFPIPLVRQKGGQYTGFEISNHDGDFIIKIPFGRWQVKKEINKHRPWEKFDFEQVRKSPKPISLLLSTQRRKRNKGWSKDEGTEAEIRKVMNGDYQTSYIEVKRGSKVGEKSAWMLNLSIDVPKIDKGVNPSIIGGIDVGVKSPLVCAINNALGRYSVSDNDLFRFNKKMFARRRILLKKNRHKRAGHGAKNKLKPITILTKKSERFRKKLIERWACEIADFFIKNKVGTVQVENLESMKRKEDSYFNIRLRGFWPYAEMQNKIEFKLKQYGIKVRKVAPNNTSKTCSKCGHLNNYFSFEYRKKNKFPHFKCEKCNFKENADYNAALNISNPKLKSTKEEP

SEQ ID NO: 1746 - protein, 726 aa, synthetic construct
SEVEFSHEYWMRYALTLARRARDEREVPVGAILVLNNRVIGEGWNRAIGLHDPTAHAEIMALRQGGLVMQNYRLTDATLYATFEPCVMCAGAMIHSRIGRVVFGVRNSKHGAAGSLMNVLNHPGMNHRVEITEGILADECAALLCDFYRMPRQVFSAQRKAQSSINFGGSSGGSSGSGTPGTSESATPESSGGSSGGSAKNTITKTLKLRIVRPYNSAEVEKIVADEKNNRERIALEKNKDKVKEACSKHLKVASYCTTQVERNACLFCKARKLDDKFYRKLRGQFPDAVFWQEIGEIFRQLQKQAAEIYNQSLIELYYEIFIKGKGFANASSVEHYLSDVCYTRAAELFKNAAIASGLRGKVKSNFRLKELKNMKSGLPTTKSDNFPIPLVKQKGGQYTGFEISSHNDDFIIKIPFGRWQVKEEIDKYRPWEKFDFEQVRKNPKPISLLLSTQRRKRNKGWSKDEGTEAEIRKVMNGDYQTSYIEVRRGSKIGEKSAWMLNLSIDVPKIDKGVDPSIIGGIDVGVKSPLVCAINNAFSRYSISDNELFHFNKKMFARRRILLKKNRHKRAGHGAKNKLKPITILTEKSGRFRKKLIERWACEIADFFIKNKVGTVQMENLESMKRKEDSYFNIRLRGFWPYAEMQNKIEFKLKQYGIEIRKVAPNNTSKTCSKCGHLNHYFNFEYRKKNKFPHFKCEKCNFKENADYNAALNISNPKLKSTKGEP

SEQ ID NO: 1747 - protein, 726 aa, synthetic construct
SEVELSHEYWMRHALTLARRARDEREVPVGAVLVLNNRVIGEGWNRAVGLHDPTAHAEIMALRQGGLVMRNYRLTDATLYVTFEPCVMCAGAMIHSRIGRVVFGVRNSKRGAAGSLMNVLNYPGMNHCVEITEGILMDECAALLCDFYRMPRQVLSAQKKAQSSINSGGSSGGSSGSETPSTSESATPESSGGSSGGSAKNTITKTLQLRIVRPYNSAEVEKIVTDEKNNREKIALEKNKDKVKEACSKHLKMASYCATQVERNACLFCKARKLDDKFYQKLRGQFPDAVFWQELGGIFRQLQKQAAEIYNQSLVELYYEIFIKGKGIANASSVEHYLSDVCYTRAAGLFKNAAIASGLRNKIKSNFRLKELRNMKSGLPTTKSDNFPIPLVRQKGGQYTGFEISNHNGDFIIKIPFGRWQVKKEISKHRPWEKFDFEQVRKSPKPISLLLSTQRRKRNKGWGKDEGTEAEIRKVMNGDYQTSYIEVKRGSKIGEKSAWMLSLSIDVPKIDKGVDPSIIGGIDVGVKSPLVCAINNAFNRYSISDNNLFHFNKKMFARRRILLKKNRHKRAGHGAKNKLKPISILTEKSERFRKKLIERWACEIADFFIRNKVGTVQMENLEGMKRREDSYFNIRLRGFWPYAEMQNKIEFKLKQYGIEVRKVAPNNTSKTCSKCGHLNNYFNFEYRKKNKFPHFKCEKCNFKENADYNAALNISNPKLKSTKEEP

SEQ ID NO: 1748 - protein, 726 aa, synthetic construct
SEVEFSHEYWMRHALTLAKRARDEREVPVGAILVLNNRVIGEGWNRAIGLNDPTAHAEIMALRQGGLVMQNYRLIDATLYVTFEPCVMCAGAMIHSRIGRVVFGVRNNKHGAAGSLMNVLNYPGMNHRVEITEGILADECAALLCDYYRMPRQVFNARKKAQSSINSGGSSDGGSGSETPGTSESATPESSGGSTGGSAKNTITKTLKLRIVRPYNSAEVEKIVADEKNNREKIALEKNKDKVKEACSEHLKVAAYCTTQVERNACLFCKARRLDDRFYQKLRGQFPDAVFWQEIGEIFRQLQKQAAEVYNQSLVELYYEIFIKGKGFANASSVEHYLSDVCYTRAAELFKNAAIASGLRGKVKSNFRLKELKNMKSGLPTTKSDNFPIPLVKQKGGQYTGFEISSHNDDFIIKIPFGRWQVKEEIDKYRPWEKFDFEQVRKNPKPISLLLSIQRRKRNKGWSKDEGTEAEIRKVMNGDYQTSYIEVKRGSKTGEKSAWMLNLSIDVPKIDKGVDPSIIGGIDVGVKSPLVCAINNAFSRYSISDNDLFRFNKKMFARRRILLKKNRHKRAGHGARNKLKPITVLTEKNERFRKKLIERWACEIANFFIKNKVGTVQMENLESMKRREDSYFNIRLRGFWPYAEMQSKIEFKLKQYGIEVRKVAPNNTSKTCSKCGHLNNYFNFEFRKKSKFPHFKCEKCNFKEDADYNAALNISNPKLKSTKEEP

SEQ ID NO: 1749 - protein, 726 aa, synthetic construct
SEVEFSHEYWMRHALTLAKRARDEREVPVGAILVLNNRVIGEGWNRAIGLHDPTAHAEIMALRQGGLVMQNYRLTDATLYVTFEPCVMCAGAMIHSRIGRVVFGVRNSKRGAAGSLMNVLNYPGMNHCVEITEGILVDECAALLCDFYRMPRRVLNAQKKAQPSISSGGSSGGSGGSETPGASESVTPKSSGGGSAGSTKNTTTKTLKLRIVRPYNSAEVEKIVADEKNNREKIALEKNKGKVKEACSKHLKVATYCTTQVERNACLFCKARKLDDKFYQKLRGQFPDAVFWQEIGEIFRQLQKQAAEIYNQSLIELYYEIFIKGKGFANASSVEHYLSDVCYTRAAELFKNAAIASGLRGKVKSNFRLKELKNMKSGLPTTKSANFPIPLVRQKGGQYTGFEISSHNDDFIIKIPFGRWQVRKEIDKYRPWEKFDFEQVRKSPKPISLLLSTQRRKRNKGWSKDEGTEAEIRKVMNGDYQTSYIEVKRGSKIGEKSAWMLNLSIDVPKIDKGVDPSIIGGIDVGVKSPLVCAIYNAFSRYSISDNDLFHFNKKMFARRRILLKKNRHKRAGHGAKNKLKPISILTEKSKRFRKKLIERWACEIADFFIKNKVGTVQMESLESMKGKEDSYFNIRLRGFWPYAEMQNKIEFKLKQYGIKIRKVAPNNTSRTCSKCGHLNNYFSFEYRKKNKFPHFKCEKCNFKENADYNAALNISNPKLKSTKEEP

SEQ ID NO: 1750 - protein, 726 aa, synthetic construct
SEVEFSHEYWMRHALTLAKRARDEREVPVGAVLVLNNRVIGEGWNRAIGLHDPTAHAEIMALRQGGLVMQNYRLTDATLYVTFEPCVMCAGAMIHSRIGRVVFGVRNSKRGAAGSLMNVLNYPGMNHCVEITEGILVDECAALLCDFYRMPRQVLSAQKKAQSSVSSGDSSGGSSGSETPGASGSVTPKSSVGSSAGSTKSTITKTLKLRIVRPYNSAEVEKIVADEKNNREKIALEKNRDKVKEACSKHLKVAAYCTTQVERNACLFCKARKLDDKFYQKLRGQFPDAVFWQEIGEIFRQLQKQAAEIYNQSLIELYYEIFIKGKGFANASSVEHYLSDVCYTRAAELFKNAAIASGLRGKVKSNFRLKELKNMKSGLPTTKSDNFPIPLVKQKGGQYTGFEISSHNDDFIIKIPFGRWQVKKEINKHRPWEKFDFEQVRKSPKPISLLLSTQRRKRNKGWSKDEGTEAEIRKVMNGDYQTSYIEVKRGSKIGEKSAWMLNLSIDVPKIDKGVDPSIIGGIDVGVKSPLVCAINNALSRYSISDNDLFHFNKKMFARRRILLRKNRHKRAGHGAKNKLKPITMMTEKSKRFRKKLIERWACEIADFFVKNKVGTVQMENLESMKRKEDSYFNIRLRGLWPYAEMQNKIEFKLKQYGIEIRKVAPNNTSKTCSKCGHLNNYFNFEYRKKNKFPHFKCEKCNFKENADYNAALNISNPKLKSTKEEP

SEQ ID NO: 1751 - protein, 726 aa, synthetic construct
SEVEFSHEYWMRHALTLAKRARDEREVPVGAVLVLNNRVIGEGWNRAIGLHDPTAHAEVMALRQGGLVMQNYRLIDATLYVTFEPCVMCAGAMIHSRVGRVVFGVRNSKHGAAGSLMNVLNYPGMNHRVEITEGILADECAALLCDFYRMPRQVFNARKKAQSSINPGGPSGGSSGSETSDTSESATPESSGGSSAGSTKNTITKTLKLRIVRPYNSAEVEKIVADEKNSREKIALEKNKDKVKEACSEHLKVAAYCTTQVERSACLFCKARKLDDRFYQKLRGQFPDAVFWQEIGEIFRQLQKQAAEIYNQSLIELYYEIFIKGKGIANASSVEHYLSDVCYTRAAELFKNAAIASGLRNKIKSNFRLKELRNMKSGLPTTKSDNFPIPLVRQKGGQYTGFEISSHNSDFIIKIPFGRWQVKEEIDKYRPWEKFDFEQVRKSPKPISLLLSTQRRKKNKGWSKDEGTEAEIRKVMNGDYQTSYIEVKRGSKIGEKSAWMLNLSIDVPKIDKGVDPSIIGGIDVGVKSPLVCAINNSSSRYSICDNDLFRFNKKMFARRRILLKKNRHKRAGHGAKNKLKPITILTEKSVRFRKKLIERWACEIADFFIKNKVGTVQMENLESMKGKEDSYFNIRLRGFWPYAEMQNKIEFKLKQYGIEIRKVAPNNTSKTCSKCGHLNNYFNFEYRKKNKFPHFKCEKCYFKEDADYNAALNISNPRLKSTKEEP

SEQ ID NO: 1752 - protein, 726 aa, synthetic construct
SEVEFSHEYWMRHALTLAKRARDEREVPVGAVLVLNNRIIGEGWNRAIGLHDPTAHAEIMALRQGGLVMQNYRLVDATLYVTFEPCVMCAGAMIHSRIGRVVFGVRNSKRGAAGSLMNVLNYPGMNHCVEITEGILVDECAALLCDFYRMPRQVLNAQKKAQSSISSGGSSGGSSCSETPGASESVTPKSSGGGSAGSTKNTITKTLKLRIVRPYNSAEVEKIVADEKNSREKIALEKNKGKVKEACSEHLKVAAYCTTQVERNACLFCKARKLDDRFYQKLRGQFPDAVFWQEIGEIFRQLQKQAAEIYNQSLIELYYEIFIKGKGFANASSVEHYLSDVCYTRAAELFKNAAIASGLRGKVKSNFRLKELKNMKSGLPTTKNDNFPIPLVKQKGGQYTGFEISSHNDDFIIKIPFGRWQVKKEIDKYRPWEKFDFEQVRKSPKPISLLLSTQRRKRNKGWCKDEGTEAEIRRVMNGDYRTSYIEVKRGSRIGEKSAWMLSLSIDVPKIDRGVDPSIIGGIDVGVKSPLVCAINNALSRYSISDNDLFRFNKKMFARRRILLKKNRHKRAGHGAKNKLKPISILTGKSERFRKKLIERWACEIADFFIKNKVGTVQMENLESMKRKEDSYFNIRLRGFWPYAEMQNKIEFKLKQYGIEIRKVAPNNTSKTCSKCGHLNNYFNFEYRKKNKFPHFKCEKCNFKENADYNAALNISNPKLKSTKEEP

SEQ ID NO: 1753 - protein, 726 aa, synthetic construct
SEVEFSHEYWMRHALTLAKRARDEREVPVGAVLVLNNRVIGEGWNRTTGLHDPTAHAEIMALRQGGLVMRNYRLTDATLYVTFEPCVMCAGAMIHSRIGRVVFGVRNSKRGAAGSLMNVLNYPGMNHCVEITEGILVDECAALLCDFYRMPRQVLNAQKKAQSSINSGCSSGGSSGSETPGTSESATPESSGGGSSGSAKNTITKTLQLRIVRPYNSAEVEKIVADEKNNREKIALEKNKGKVKEACSKHLRVASYCTTQVERNACPFCKARKLDDKFYQKLRGQFPDAVLWQELGEILRQLQKQAAEIYNQSLIELYYEIFIKGRGFANASSVEHYLSDVCYTRAAELFKNAAIASGLRGKVKSNFRLKELKNMKSGLPTTKSDNFPIPLVKQKGGQYTGFEISSHNDDFIIKIPFGRWQVKKEIDKYRPWEKFDFEQVRKSPKPISLLLSTQRRKRNKGWSKDEGTEAEIRKVMNGDYQTSYIEVKRGSKTGEKSAWMLNLSIDVPKIDKGVDPSIIGGIDVGVRSPLVCAINNAFSRYSISDNDLFRFNKKMFARRRILLKKNRHRRAGHGAKNKLKPISILTGRSERFRKKLIERWACEIADFFIKNKVGTVQMENLESMKRKEDSYFNIRLRGFWPYAEMQNKIEFKLKQYGIEIRKVAPNNTSKTCSKCGHLNNYFNFEYRKKNKFPHFKCEKCNFKENADYNAALNISNPKLKSTKEEP

SEQ ID NO: 1754 - protein, 726 aa, synthetic construct
SEVEFSHEYWMRHALTLAERARDEREVPVGAVLVLNNRVIGEGWNRAIGLHDPTAHAEIMALRQGGLVMQNYRLTDATLYVTFEPCVMCAGAMIHSRIGRVVFGVRNSKRGAAGSLMNVLNYPGINHCVEITEGILVDECAALLCDFYHMPRQVLNAQKKAQSSISSGGSSGGSSGSETPGASESVTPKSSVGSSAGSTKNTITKTLKLRIVRPYNSAEVEKIVADEKDNREKIALEKNKDKVKEACSKHLKVAAYCTTQVERNACLFCKARKLDDKFYQKLRGQFPDAVFWQEVGEIFRQLQKQAAEIYNQSLVELYYEIFIKGKGFANASSVEHYLSDVCYTRAAELFKNAAIASGLRGKVKSNFRLKELKNMKSGLPTTKSGNFPIPLVKQKGGQYTGFEISSHNDDFIIKIPFGRWQVKKEIDKYRPWEKFDFEQVRKSPKPISLLLSTQRRKRNKGWSKDEGTEAEIRKVMNGDYQTSYIEVKRGSKIGEKSAWMLNLSIDVPKIDKGVDSSIIGGIDVGVKSPLVCAINNAFSRHSISDNDLFHFNKKMFARRRILLKKNRHKRAGHGAKNKLKPITILTEKSGRFRKKLIERWACEIADFFIKNKVGTVQMENLESMKRKEDSYFNIRLRGFWPYAEMQNKIEFKLKQYGIEIRKVAPNNTSKTCSKCGHLNNYFNFEYRKKNKFPHFKCEKCNFKENADYNAALNISNPKLKSTKEEP

SEQ ID NO: 1755 - protein, 726 aa, synthetic construct
SEVEFSHEYWMRHALTLAKRARDEREVPVGAVLVLNNRVIGEGWNRAIGLHDPTAHAEIMALRQGGLVMQNYRLTDATLYVTFEPCVMCAGAMIHSRIGRVVFGVRNSKRGAAGSLMNVLNYPGMNHCVEITEGILVDECAALLCDFYRMPRQVLNAQKKAQSSISSGGSSGGSSGSETPGASGSVIPKSSGGSSAGSTKDTITKTLKLRIVRPYNSAEVEKIVADEKNSREKIALEKNKGKVKEACSEHLKVAAYCTTQVERSACPFCKARKLDDRFYQKLRGQFPDAVFWQEISEIFRQLQKQAAEIYNQSLIELYYEIFIKGKGFANASSVEHYLSDVCYTRAAELFKNAAIASGLRGKVKSNFKLKELKSMKSGLPSTRSDNFPIPLVKQKGGQYTGFEISSHNDDFIIKVPFGRWQVKKEIDKYRPWEKFDFEQVRKSPKPISLLLSTQRRKRNKGWSKDVGTEAEIRKVMNGDYQTSYIEVKRGSKIGEKSAWMLNLSIDVPKIDKGVDPSIIGGIDVGVKSPLVCAINNAFSRYSISDNDLFRFNKKMFARRRILLKKNRHQRAGHGAKNKLKPITILTEKSGRFRKKLIERWACEIADFFIKNKVGTVQMENLESMKRKEDSYFNIRLRGFWPYAEMQNKIEFKLKQYGIKIRKVAPNNTSKTCSKCGHLNNYFSFEYRRKNKFPHFKCEKCNFKEDADYNAALNISNPKLKSTKEEP

SEQ ID NO: 1756 - protein, 726 aa, synthetic construct
SEVEFSHEYWMRHALTLAKRARDEREVPVGAVLVLNNRVIGEGWNRAIGLHDPTAHAEIMALRQGGLVMQNYRLIDATLYVTFEPCVMCAGAMIHSRIGRVVFGVRNSKHGAAGSLVNVLNYPGMNHRVEITEGILADECAALLCNFYRMPRQVFNVRKKAQSSINPGGSSGGSSGSETPGTSESATPESSGGSPGGSARNTITKTLKLRIVRPYNSAEVEKIVADEKNSREKIALEKNKDKVKEACSEHLKVAAYCTTQVERNACLFCKARKLDDGFYQKLRGQFPDAVFWQEIGEIFRQLQKQAAEIYNQSLIELYYEIFIKGKGFANASSVEHYLSDVCYTRAAELFKNAAIASGLRGKVKSNFRLKELKNMKSGLPTTKSDNFPIPLVKQKGGQYTGFEISSHNDDLIVKIPFGRWQVKKEIDRYRPWEKFDFEQVRKSPKPISLLLSTQRRKRNKGWSKDEGTEAEIKKVMNGDYQISYIEVKRGSKIGEKSAWTLNLSVDVPKIDKGVDPSIIGGIDVGVKSPLVCAINNALSRYSISDNDLFHFNKKVFARRRILLKKNRHRRAGHGAKNKLKPITILTEKSKRFRKKLIERWACEIADFFIKNKVGIVQMENLESMKRKEDSYFNIRLRGLWPYAEMQNKIEFKLKQYGIEIRKVAPNNTSKTCSKCGHLNNYFNFEYRKTNKFPYFKCEKCNFKEDADYNAALNISNPKLKSTKEEP

SEQ ID NO: 1757 - protein, 726 aa, synthetic construct; identical to SEQ ID NO: 684

SEQ ID NO: 1758 - protein, 726 aa, synthetic construct
SEAEFSHEYWMRHALTLAKRARDEREVPVGAVLVLNNRVIGEGWNRAIGLHDPTAHAEIMALRQGGLVMQNYRLIDATLYVTFEPCVMCAGAMIHSRIGRVVFGVRNSKHGAAGSLMDVLNYPGMNHRVEITEGILADECAALLCDFYRMPRQVFSARKKAQSSINPGGSSGGSSGSKTPGTSESATPESSGGSSGGSARNTITKTLQLRIVRPYNSAEVEKIVTDEKNNREKIALEKNKDKVKEACSKHLKMASYCTTQVERNACLFCKARKLDDKFYQKLGGQFPDAVFWQELGEIFRQLQKQAAEIYNQSLIELYYEIFIKGKGLANASSVEHYLSDVCYTRAAELFKNAAIASGLRGKVKSNFKLKELKSMKSGLPSTKSDNFPIPLVKQKGGQYTGFEIRGHNDDLIIKIPFGRWQVKKEIDKYRPWEKFDFEQVRKSPKPISLLLSTQRRKRNKGWSKDEGTEAEIRKVMNGDYQTSYIEVKRGSKIGEKSAWMLNLSIDVPKIDKGVDPSVIGGIDVGVKSPLVCAINNAFSRFSISDNDLFHFNKKMFARRRILLKRNRHKRAGHGAKNKLKPISILTEKSKRFRKKLIERWACEIADFFIKNKVGTVQMENLESMKRREDSYFNIRLRGFWPYAEMQNKIEFKLKQYGIEIRKVAPNNTSKTCSKCGHLNNYFNFEYRKMNKFPHFKCEKCNFKENADYNAALNISNPKLKSTKEEP

SEQ ID NO: 1759 - protein, 726 aa, synthetic construct
SEVEFSHEYWMRHALTLAKRARDGREVPVGAVLVLNNRVIGEGWNRAIGLHDPTAHAEIMALRQGGLVMQNYRLIDATLYVTFEPCAMCAGAMVHSRIGRVVFGVRNSKRGAAGSLMNVLNYPGMDHRVEITGGILADECAALLCDFYRMPRRVFNAQKKAQSSINSGGSSGGSSGSVTPDTSESATPESSGGSFGGSAKNTITKTLQLRIVRPYNSAEVEKIVADEKNNREKVALEKNKDKVKEACSKHLKVASYCTTQVERNACLFCKARKLDDKFYQKLRGQFPDAVFWQEIGEIFRQLQKQAAEIYNQSLIELYYEIFIKGKGFANASSVEHYLSDVCYTRAAELFKNAAIASGLRGKVKSNFRLKELKNMRSGLPTTKSDNFPIPLVKQKGGQYTGFEISDHNSDFIIKIPFGRWQAKKEIDKYRPWEKFDFEQVRKSPKPISLLLSTQRRKKNRGWSKDEGTEAEIKKVMNGDYQTSYIEVKRGSKIGEKSAWMLNLSIDVPKIDKGVDPSIVGGIDVGVKSPLVCAISNAFSRYSISDNDLFRFNKKVFARRRILLKKNRHKRAGHGTKNKLKPITILTEKSGRFRKKLIERWACEIANFFVKNKVGTVQMEDLESMKRKEDSYFNIRLRGFWPYAEMQNKIEFKLKQYGIKIRKVAPNNTSKTCSKCGHLNNYFNFEYRKKNKFPHFKCEKCNFKEDADYNAALNISNPKLKNTKGEP

SEQ ID NO: 1760 - protein, 726 aa, synthetic construct
SEVEFSHEYWMRHALTLAKRARDEREVPVGAVLVLNNRVIGEGWNRAIGLHDPTAHAEIMALRQGGLVMQNYRLTDATLYVTFEPCVMCAGAMIHSRIGRVVFGVRNSKRGAAGSLMNVLNYPGMNHRVEITEGILVDECAALLCDFYHMPRQVLNAQKKAQSSISSGGSSGGCSGSEMPGASESVTPKSSGGSSAGSTKNTITKTLKLRIVRPYNSAEVEKIVADEKNNREKIALEKNKDKVKEACSKHLKVAAYCTTQVERNACQFCKARKLDDKFYQKLRGQFPDAVFWQEIGEIFRQLQKQAAEIYNQSLIELYYEIFIKGKGFANASSAEHYLSDVCYTRAAELFKNAAIASGLRGKVKSNFRLKELKNMKSGLPTTKSDNFPIPLVKQKGGKYTGFEISSHNDDFIIKIPFGRWQVKKEIDKYRPWEKFDFEQVRKSPKPISLLLSTQRRKRNKGWSKDEGTEAEIRKVMNGDYQTSYIEVKRGSKIGEKSAWMLNLSIDVPKIDKGVDPSIIGGIDVGVKSPLVCAINNAFGRYSISDNELFHFNKKMFARRRILLKKNRHKRAGHGAKNKLKPISTLTERSKRFRKKLIERWACEIADFFIKNKVGTVQMENLESMKRKEDSYFNIRLRGFWPYAEMQNKIEFKLKQYGIEIRKVAPNNTSKTCSKCGHLNNYFNFEYRKKNKFPHFECEKCNFKENADYNAALNISNPKLKSTKKEP

SEQ ID NO: 1761 - protein, 726 aa, synthetic construct
SEVEFSHEYWMRHALTLAERARDEREVPVGAVLVLNNRVIGEGWNRTTGLHDPTAHAEIMALRQGGLVMRNYRLTDATLYVTFEPCVMCAGAMIHSRIGRVVFGVRNSKRGAAGSLMNVLNYPGMNHRVEITEGILVDECAALLCDFYRMPRQVLNAQKKAQSSISPGGSSGGSSGSETPGASESVTPKSSGGSSGGSAKNTITKTLKLRIVRPYNSAEVEKIVADEKNNREKIALEKNKDKVKEACSEHLKVAAYCTTQVERNACLFCRARKLDDKFYQKLRGQFPDAVFWQEIGEIFRQLQKQAAEIYNQSLIELYYEIFIKGKGFANASSVEHYLSDVCYTRAAELFKNAAIASGLRGKVKSNLRLKELKNMKSGLPTTKSDNFPIPLVKQKGGQYAGFEISSHNDDFIIKIPFGRWQVKKEIDKYRPWEKFDFEQVRKSPKPISLLLSTQRRKRNKGWGKDEGTEAEIRKVMNGDYQTSYIEVKRGSKIGEKGAWMLSLSIDVPKIDKGVDPRIIGGIDVGVKSPLVCAINNAFSRYSISDNDLFHFNKKMFARRRILLKKNRHKRAGHGAKNKLKPITILTEKSVRFRKKLIERWACEIADFFIKNKVGTVQMENLESMKGKEDSYFNIRLRGFWPYAEMQNKIEFKLKQYGIGIRKVAPNNTSKTCSKCGHLNNYFNFEYRKKNKFPHFKCEKCYFKEDADYNAALNISNPRLKGTKEVP

SEQ ID NO: 1762 - protein, 726 aa, synthetic construct
SEVEFSHEYWMRRALTLAKRARDEREVPVGAVLVLNNRVIGVGWNRAAGLHDPTAHAEIMALRQGGLVMQNYRLANATLYVTFEPCVMCAGAMIHSRIGRVVFGVRNSKRGAAGSLMNVLNYPGMNHRVEITEGILTDECAALLCDFYRMPHQVFNARKKAQPSINPGGSSGGSSGSETPGTSESATPESSGGSSGGSAKNTITKTLKLRIVRPYNSAEVEKIVADEKNNREKIALEKNKDKVKEACSKHLKVASYCTTQVERNACLFCKARKLDDKFYQKLRGQFPDAVFWQELGEIFRQLQKQAAEIYNQSLIELYYEIFIKGKGLANASSVEHYLSDVCYTRAAELFKNAAIASGLRGKVKSNFRLKELKSMKSGLPSTKSDNFPIPLVKQRGGQYTGFEISSHNDDFIIKIPFGRWQAKKEIDKYRPWEKFDFEQVRKSPKPISLLLSTQRRKRNKGWSKDEGTEAEIRKVMDGDYQTSYIEVKRGSKIGEKSAWMLNLSIDVPKIDKGVDPSIVGGIDVGVKSPLVCAIDNALSRYSISDNDLFHFNKKMFARRRILLKKNRHRRAGHGAKNKLKPISILTEKSKRFRKKLIERWACEIADFFIKNKVGTVQMENLESMKRKEDSYFNIRLRGFWPYAEMQNKIEFKLKQYGIEIRKVAPNNTSKTCSKCGHLNNYFSFEYRKKNKFPHFKCEKCNFKENADYNAALNISNPKLKSTKEEP

SEQ ID NO: 1763 - protein, 726 aa, synthetic construct
SEVEFSHEYWMRRALTLAKRARDEREVPVGAVLVLNNRVIGVGWNRAVGLHDPTAHAEIMALRQGGLVMQNYRLIEATLYVTFEPCIMCAGAMIHSRIGRVVFGVRNSKRGAAGSLVNVLNYPGMNHRVEITEGILVDECAALLCDFYRMPRQVFNAQKKAQSTINSGGSSGGSSGSETPGTSESPTPESSGGSSGGSAKNTITKTLKLRIVRPYNSAEVEKIVADEKNNREKIALEKNKDKVKEACSKHLKVAAYCTTQVERNACLFCKARKLDDKFYQKLRGQFPDAVFWQEIGEIFRQLQKQAAEIYNQSLIELYYEIFIKGKGFANASSVEHYLSDVCYTRAAELFKNAAIASGLRGKVKSNFRLKELKNMKSGLPTTKSDNFPIPLVKQKGGQYTGFEISSHNDDFIIKIPFGRWRVKKEIDKYRPWEKFDFEQVRKSPKPISLLLSTQRRKRNKGWSKDEGTEAEIRKVMNGDYRTSYIEVKRGGKTGEKSAWVLNLSIDVPKIDKGVDPSIIGGIDVGVKSPLVCAINNAFSRYSISDNDLFRFNKKMFARRRILLKKNRHKRAGHGAKNKLKPISILTGKSERFRKKLIERWACEIADFFIKNKVGTVQMENLESMKKKEDSYFNIRLRGFWPYAEMQNRIEFKLKQYGIEIRKVAPNNTSKTCSKCGHLNNYFNFEYRKKNKFPHFKCEKCNFKENADYNAALNISNPKLKSTKEEP

SEQ ID NO: 1764 - protein, 726 aa, synthetic construct
SEVEFSHEYWMRHALTLAKRARDEREVPVGAILVLNNRVIGEGWNRAIGLNDPTAHAEIMALRQGGLVMQNYRLIDATLYVTFEPCVMCAGAMIHSRIGRVVFGVRNNKHGAAGSLVNVLNYPGMNHRVEITEGVLADECAALLCDFYRMPRQVFNARKKAQSSINPGGSSGGSGGSETPGTSESATPESSGGSSGSSAKNTITKTLKLRIVRPYNSAEVEKIVADEKNNREKIALEKNKDKVKEACSKHLKVATYCTTQVERNACLFCKARRLDDKFYQKLRGQFPDAVFWQEIGEIFRQLQKQAAEIYNQSLVELYYEILIKGKGIANASSVEHYLSDVCYTRAAELFKNAAIASGLRNKIKSNFRLKELRNMKSGLPTTKSDNFPIPLVRQKGGQYTGFEISNHDGDFIIKIPFGRWQVKKEINKHRPWEKFDFEQVRKSPKPISLLLSTQRRKKNRGWSKDESTEAEIKKVMNGDYQTSYIEVKRGSKVGEKSAWMLNLSIDVPKIDKGVDPSIIGGIDVGVKSPLVCAINNAFSRYSISDNDLYRFNKKMFARRRILLKKSKHKRAGHGAKNKLKPITILTEKSGRFRKKLIERWACEIADFFIKNKVGTVQMENLEGMKRKEDSYFNIRLRGFWPYAEMQNKIEFKLKQYGIEIRKVAPNNTSKTCSKCGHLNNYFNFEYRKKNKFPHFKCEKCNFKENADYNAALNISNPKLKSTKEEP

SEQ ID NO: 1765 - protein, 726 aa, synthetic construct
SEVEFSHEYWMRHALTLAKRARDEREVPVGAILVLNNRVIGEGWNRAIGLHDPTAHAEIMALRQGGLVMQNYRLIDATLYVTFEPCVMCAGAMIHSRIGRVVFGVRNNKHGAAGSLVNVLNYPGMNHRVEVTEGILADECAALLCDFYRMPRQVFNARKKAQSSINPGGSSGGSSGSETPGTSESATPESSGGSSGSSAKNTITKTLKLRIVRPYNSAEVEKIVADEKNNREKIALEKSKDKVKEACSKHLKVASYCTTQVERNACLFCKARKLDDKFYQKLRGQFPDAVFWQELGGIFRQLQKQAAEIYNQSLIELYYEIFIKGKGITNASRVEHYLSDVCYTRAAELFKNAAIASGLRSKVRSNFRLKELKNMKSGLPTTKSDNFPIPLVKQKGGQYTGFEISSHNSDFIIKIPFGRWRVKEEIDKYRPWEKFDFEQVRKSPKPISLLLSTQRRKKNKGWSKDEGTEAEIRRVMNGDYQTSYIEVKRGSKIGEKSAWMLNLSIDVPKIDRGVDPSIIGGIDVGVKSPLVCAINNAFGRYSISDNDLFRFNKKMFARRRILLKKNRHKRAGHGAKNKLKPITILTGKSERFRKKLIERWACEIADFFIKNKVGTVQMENLEGMKRKEDSYFNIRLRGLWPYAEMQNKIEFKLKQYGIEIRKVAPNNTSKTCSKCGHLNNYFNFEYRKKNKFPHFKCEKCNFKENADYNAALNISNPKLKSTKEEP

SEQ ID NO: 1766 - protein, 726 aa, synthetic construct
SEVEFSHEYWMRHALTLAKRARDEREVPVGAVLVLDNRVIGEGWNRAIGLYDPTAHAEIMALRQGGLVMQNYRLTDATLYVTFEPCVMCAGAMIHSRIGRVVFGVRNSKRGAAGSLMNVLNYPGMNHCVEITEGILVDECAALLCDFYRMPRQVLNAQKKAQSSISSGGSSGGSSCSETPGASESVTPKSSGGSSAGSTKNTITKTLKLRIVRPYNSAEVEKIVADEKNSREKIALEKNKDKVKEACSKHLKVATYCTTRVERNACLFCKARKLDDKFYQKLRGQFPDAVFWQEVGEIFRQLQKQAAEIYNQSLIELYYEIFIKGKGFANASSVEHYLSDVCYTRAAELFKNAAIASGLRGKVRSNFRLKELRNMKSGLPTTKSDNFPIPLVKQKGGQYTGFEISSHNDDFIIKIPFGRWQVKEEIDKYRPWEKFDFEQVRKNPKPISLLLSTQRRRRNKGWSKDEGTEAEIRKVMNGDYQTSYIEVKRGSKIGEKSAWMLNLSIDVPKIDKGVNPSIIGGIDVGVKSPLVCAINNSSSRYSICDNDLFRFNKKMFARRRILLKKNRHKRAGHGAKNKLKPITILTEKSGRFRKKLIERWACEIADFFVKNKVGTVQMENLESMKRKEDSYFNIRLRGFWPYAEMQNKIEFKLKQYGIKVRKVAPNNTSKTCSKCGHLNNYFNFEYRKKNKFPHFKCEKCNFKENADYNAALNISNPKLKSTKEEP

SEQ ID NO: 1767 - protein, 726 aa, synthetic construct
SEVEFSHEYWMRHALTLAKRARDEREVPVGAVLVLNNRVIGEGWNRAIGLHDPTAHAEIMALRQGGLVMQNYRLIDATLYVTFEPCVMCAGAMIHSRIGRVVFGVRNNKHGAAGSLVNVLNYPGMNHRVEITEGILADECAALLCDFYRMPCQVFNARKKAQSSISPGGPSGGSSGSETPGTSESAAPESSGGSSGGSAKNTITKTLKLRIVRPYNSAEVEKIVADEKNNREKIALEKNKDKVKEACSKHLKVASYCTTQVERSACPFCKARKLDDKFYQKLGGQFPDAVFWQELGEILRQLQKQAAEIYNQSLIELYYEIFIKGRGFANASSVEHYLSDVCYTRAAELFKNAAIASGLRGKVKSNFRLKELKNMKSGLPTTKSDNFPIPLVKQKGGQYTGFEISSHNDDFIIKIPFGRWQVKREIDKYRPWEKFDFEQVRKSPKPISLLLSTQRRKRNKGWSKDEGTEAEIKKVMNGDYQISYIEVKRGSKIGEKSAWTLNLSVDVPKIDKGVDPSIIGGIDVGVKSPLVCAINNALSRYSISDNDLFHFNKKVFARRRILLKKNRHRRAGHGAKNKLKPITILTEKSKRFRKKLIERWACEIADFFIKNKVGIVQMENLESMKRREDSYFNIRLRGFWPYAEMQNKIEFKLKQYGIGIRKVAPNNTSKTCSRCGHLNNYFNFEHRKKNKFPRFKCEKCNFKENADYNAALNISNPKLKSTKEEP

SEQ ID NO: 1768 - protein, 726 aa, synthetic construct
SEVEFSHEYWMRHALTLAKRARDEREVPVGAILVLNNRVIGEGWNRAIGLHDPTAHAEIMALRQGGLVMQNYRLIDATLYVTFEPCVMCAGAMIHSRIGRVVFGVRNNKHGAAGSLVNVLNYPGMNHRVEITEGILADECAALLCDFYRMPRQVFSARKKAQSSINPGGSSGGSSGSETPGASESATPESSGGSSGGSAKNTITKTLKLRIVRPYNSAEVEKIVADEKNNREKIALEKNKDKVKEACSKHLKVAAYCTTQVERNACPFCKARRLDDKFYQKLRGQFPDAVFWQEIGEIFRQLQKQAAETYNQSLIELYYEIFIKGKGIANASNVEHYLSDVCYTRAAELFKNAAIASGLRNKIKSNFRLKELRNMKSGLPTTKSDNFPIPLVRQKGGQYTGFEISNHNSDFIIKIPFGRWQAKKEIDKYRPWEKFDFEQVRKSPKPISLLLSTQRRKRNKGWSRDEGTEAEIRKVMNGDYQVSYIEVKRGSKIGEKSAWMLNLSIDVPKIDKGVDPSIIGGIDVGVKSPLVCAINDAFSRYSISDNDLFRFNKKMFARRRILLKKNRHKRAGHGAKNKLKPISILTGKSERFRKKLIERWACEIADFFIKNKVGTVQMENLESMKRKEDSYFNIRLRGFWPYAEMQNKIEFKLKQYGIEIRKVAPNNTSKTCSKCGHLNNYFNFEYRKKNKLPHFKCEKCNFKEDADYNAALNISNPKLKSTKEEP

SEQ ID NO: 1769 - protein, 726 aa, synthetic construct
SEVEFSHEYWMRHALSLAKRARDAREVPVGAILVLNNRVIGEGWNRAIGQHDPTAHAEIMALRQGGLVMQNYRLIDATLYVTFEPCVMCAGAMIHSRIGRVVFGVRNSKHGAAGSLMNVLNYPGMNHRVEITEGILADECAALLCDFYRMPRQVFNGRKKAQSSNNSGGSSGGSSGSETPGTSESPTPESSGGSPGGSAKNTITKTLKLRIVRPYNSAEVEKIVADEKNNREKIAVEKNKDKVKEACSKHLKVAAYCTTQVERNACLFCKARKLDDKFYQKLRGQFPDAVFWQEIGEIFRQLQKQAAEIYNQSLIELYYEIFIKGKGFANASSVEHYLSDVCYSRAAELFKNAAIASGLRGKVKSNFRLKELKNMKSGLPTTKSDNFPIPLVKQKGGQYTGFEISSHDDDFIIKIPFGRWQVKEEIDKYRPWEKFDFEQVRKNPKPISLLLSTQRRKGNKGWSKDEGTEAEIRKVMNGDYQTSYIEVKRGSKIGEKSAWMLNLSIDVPKIDKGVDPSIIGGIDVGVKSPLVCAINNAFCRYSISDNDLFHFNKKMFARRRILLKKSRHKRAGHGAKNKLKPISILTEKSKRFRKKLIERWACEIADFFIKNKVGTVQMENLESMKRKEDSYFNIRLRGFWPYAEMQNKIEFKLKQYGIEIRKVAPNNTSKTCSKCGHLNNYFNFEYRKKNKFPHFKCEKCSFKENADYNAALNISNPKLKSTKEEP

SEQ ID NO: 1770 - protein, 726 aa, synthetic construct
SEVEFSHEYWMRHALTLAKRARDEREVPVGAVLVLNNRVIGEGWNRAIGLHDPTAHAEIMALRQGGLVMQNYRLTDATLYVTFEPCVMCAGAMIHSRIGRVVFGVRNSKRGAAGSLMNVLNYPGMNHCVEITEGILVDECAALLCDFYRMPRQVLNAQKKAQSSINPGGSSGGSSCSETPGASESVTPKSSGGSSTGSTKNTITKTLKLRIVRPYNSAEVEKIVADEKNSREKIALEKNKGKVKEACSEHLKVAAYCTTQVGRNACLFCKARKLDDRFYQKLRGQFPDAVFWQEIGEIFRQLQKQAAEIYNQSLIELYYEIFIKGKGFANASSVEHYLSDVCYTRAAELFKNAAIASGLRGKVKSNFRLKELKNMKSGLPTTKSDNFPIPLVKQKGGQYTGFEISSHNDDFIIKIPFGRWQVRKEIDKYRPWEKFNFEQVRKSPKPISLLLSTQRRKRNKGWSRDEGTEAEIRKVMNGDYQTSYIEVKRGSKIGEKSAWMLNLSIDVPKIDKGVDPSIIGGIDVGVKSPLVCAINNAFSRYSISDNELFHFNKKMFARRRILLKKNRHKRAGHGTKNKLKPITILAEKSGRFRKKLIERWACEIANFFIKNKVGTVQMENLESMKRKEDSYFNIRLRGFWPYAEMQNKIEFKLKQYGIEIRKVAPNNTSKTCSKCGHLNNYFNFEYRKMNKFPHFKCEKCNFKENADYNAALNISNPKLKSTKEEP

SEQ ID NO: 1771 - protein, 726 aa, synthetic construct
SEVEFSHEYWMRHALTLARRARDEREVPVGAILVLNNRVIGEGWNRAIGLHDPTAHAEIMALRQGGLVMQNYRLIDATLYVTFEPCVMCAGAMIHSRIGRVVFGVRNSKHGAAGSLVNVLNYPGMNHRVEITEGILADECAALLCDFYRMPRQVFNARKKAQSSINSGGSSGGSSGSDTPGTSESATPESSGGGSSGSAKNTITKTLQLRIVRPYNSAEVEKIVADEKNNREKIALEKNKDKVREACSKHLKVASYCTTQVERNACPFCKARKLDDKFYQKLRGQFPDAVFWQELGEILRQLQKQAAEIYNQSLIELYYEIFIKGRGFANASSVEHYLSDVCYTRAAELFKNAAIASGLRNKIKSNFRLKELRNMKSGLPTTKSDNFPIPLVRQKGGQYTGFEISNHNGDFIIKIPFGRWQVKKEISKHRPWEKFDFEQVRKSPKPISLLLSTQRRKRNKGWGKDEGTEAEIRKVMNGDYQTSYIEVKRGSKVGEKSAWMLNLSIDVPKIDKGVDPSIIGGIDVGVRSPLVCAINNALSRYSISDNDLFHFNKKMFARRRILLRKNRHKRAGHGARNKLKPITVLTEKSERFRKKLIERWACEIANFFIKNKVGTVQMENLESMKRREDSYFNIRLRGFWPYAEMQSKIEFKLKQYGIKIRKVAPNNTSKTCSKCGHLNNYFNFEFRKKNKFPHFKCEKCNFKEDADYNAALNISNPKLKSTKEEP

SEQ ID NO: 1772 - protein, 726 aa, synthetic construct
SEVEFSHEYWMRHALTLAKRARDEREVPVGAVLVLNNRVVGEGWNRAIGLHDPTAHAEIMALRQGGLVMQNYRLTDATLYVTFEPCVMCAGAMIHSRIGRVVFGVRNSKRGAAGSLMNVLNYPGMNHCVEITEGILVDECAALLCDFYRMPRQVLSAQKKAQSSISSGGSSGGSSGSETPGASGSVTPKSSVGSSAGSTKNTITKTLKLRIVRPYNSAEVEKIVADEKNNREKIALEKNKDKVKEACGKHLKMASYCTTQVERNACLFCKARKLDDKFYQKLRGQFPDAVFWQELGGIFRQLQKQAAEIYNQSLIELYYEIFIKGKGITNASRVEHYLSDVCYTRAAELFKNAAIASGLRSKVRSNFRLKELKNMKSGLPTTKSDNFPIPLVKQKGGQYTGFEISNHNSDFIIKIPFGRWQVKKEIDKYRPWEKFDFEQVRKSPKPISLLLSTRRRKRNKGWSKDEGTEAEIRKVMNGDYQTSYIEVKRGSKTGERSAWMLNLSIDVPKIDKGVNPSIIGGIDVGVKSPLVCAINNAFSRYSISDNDLFRFNKKMFARRRILLGKNRHKRAGHGVKNKLKPITILTEKSGRFRKKLIERWACEIADFFIKNKVGTVQMENLESMKRKEDSYFNIRLRGFWPYAEMQNKIEFKLKQYGIVVRKVAPNNTSKTCSQCGHLNNYFNFEYRKKNKFPYFKCEKCNFKENADYNAALNISNPQLKSTKGEP

SEQ ID NO: 1773 - protein, 726 aa, synthetic construct
SEVEFSHEYWMRHALTLAKRARDEREVPVGAVLVLNNRVIGEGWNRAIGLHDPTAHAEIMALRQGGLVLQNYRLADATLYVTFEPCVLCAGAMVHSRIGRVVFGARNSKRGAAGSLMNILNYPGMNHRVEITEGILADECAALLCDFYRMPRQVFNAQKKAQSSINSGGSSGGSSGSETPGTSESATPESSGGSSGGSAKNTITKTLKLRIVRPYNSAEVEKIVANEKNNREKIALEKNKDKVKEACSKHLKVASYCTTQVERNACLFCKARKLDDKFYQKLRGQFPDAVFWQELGEILRQLQKQAAEIYNQSLIELYYEIFIKGRGFANAGSVEHYLSDVCYTRAAELFKNAAIASGLRGKVKSNFRLKELKNMKSGLPTTKSDNFPIPLVKQKGGQYTGFEISSHNDDFIIKIPFGRWQVKKEIDKYRPWEKLDFEQVRKSPKPISLLLSTQRRKRNKGWSKDEGTEAEIRKVMNGDYQTSYIEVKRGSKTGEKSAWMLNLSIDVPKIDKGVDPSIIGGIDVGVKSPLVCAINNAFSRYSISDNDLFRFNKKMFARRRVLLKKNRHKRAGHGAKNKLKPISILTGKSERFRKKLIERWACEIADFFIKNKVGTVQMENLESMKRKEDSYFNIRLRGFWPYAEMQNKIEFKLKQYGIEIRKVAPNNTSKTCSKCGHLNNYFNFEYRKKNKFPHFKCEKCNFKENADYNAALNISNPKLKSTKEEP

SEQ ID NO: 1774 - protein, 726 aa, synthetic construct
SEVEFSHEYWMRHALTLAKRARDEREVPVGAVLVLNNRVIGEGWNRAIGLHDPTAHAEIMALRQGGLVMQNYRLTDATLYATFEPCVMCAGAMIHSRIGRVVFGVRNSKHGAAGSLMNVLNYPGMNHRVEITEGILADECAGLLCDFYRMPRQVFSARKKAQSSINPGGSSGGSSGGKAPGTSESATLESSGGSSGGSAKNSITKTLKLRIVRPYNSAEVEKIVADEKNNREKTALEKNKDKVKEACSKHLKVATYCTTQVERNACLFCKARKLDDKFYQKLRGQFPDAVFWQEIGEIFRQLQKQAAEIYNQSLIELYYEIFIEGKGSANARSVEHYLSDVCYTRAAELFKNAAIASGLRGKVKGNFRLKELKSMKSGLPTTKSDNFPIPLVKQKGGQYTGFEISSHNDDFIIKIPFGRWQVKKEIDKYRPWEKFDFEQVRKSPKPISLLLSTQRRKRNKGWSKDEGTEAEIRKVMNGDYQISYIEVKRGSKIGEKSAWMLSLSIDVPKIDKGVDPSIIGGIDVGVRSPLVCAIDNAFSRYSISDNDLFHFNKKMFARRRILLKKNRHKRVGHGAKNKLKPISILTEKSKRFRKKLIERWACEIADFFIKNKVGTVQMENLVSMKRKEDSYFNIRLRGLWPYAEMQNKIEFKLKQYGIKIRKVAPNNTSKTCSKCGHLNNYFNFEYRKKNKFPHFKCEKCSFKENADYNAALNISNPKLKSTKEEP

SEQ ID NO: 1775 - protein, 726 aa, synthetic construct
SEVEFSHEYWMRHALTLAKRARDEREVPVGAVLVLNNRVIGEGWNRAIGLHDPTAHAEIMALRQGGLVMQNYRLTDATLYVTFEPCVMCAGAMIHSRIGRVVFGVRNSKRGAAGSLMNVLNYPGMNHCVEITEGILVDECAALLCDFYRMPRQVLNAQKKAQSSISSGGSSGGSSGSETPGASESPTPESSGGSSGGSAKNTITKTLQLRIVRPYNSAEVEKIVADEKNNREKIALEKNKDKVKEACSKHLKVASYCTTQVERNACPFCKARKLDDKFYQKLRGQFPDAVFWQEIGEIFRQLQKQAAEIYNQSLIELYYEIFIKGKGFANASSVEHYLSDVCYTRAAELFKNAAIASGLRSKVRSNFRLKELKNMKSGLPTTKSDNFPIPLVKQKGGQYTGFEISSHNSDFIIKIPFGRWQVKEEIDKYRPWEKFDFEQVRKSPKPISLLLSTQRRKRNRGWSKDEGTEAEIKKVMNGDYQTSYIEVKRGSKTGGKSAWMLNLSIDVPKIDKGVDPCIIGGIDVGVKSPLVCAINDAFSRYSISDNDLFHFNKKMFARRRILLKKNRHKRAGHGAKNKLKPITIMTEKSKRFRKKLIERWACEIADFFIKNKVGTVQMENLESMKRKEDSYFNIRLRGFWPYAEMQNKIEFKLKQYGIEIRKVAPNNTSKTCSKCGHLNYYFNFEYRKKNKFPHFKCEKCNFKEDADYNAALNISNPKLKSTKEEP

SEQ ID NO: 1776 - protein, 726 aa, synthetic construct
GEDEFSHEYWMRHALTLAKRARDGREVPVGAVLVLNNRVIGEGWNRAIGLHDPTAHAEIMALRQGGLVMQNYRLIDATLYVTFEPCIMCAGAMIHSRIGRVVFGVRNSKRGAAGSLMNVLNYPGMNHRVEITEGVLADECAALLCDFYRMPRQVLNAQKKAQSSINSGGSSGGSSSSETPGTSESATPESSGGSSGGSAKNTITKTLKLRIVRPYNSAEVEKIVADEKNNREKIALEKNKDKVKEACSKHLKVAAYCTTQVERNACLFCKARKLDDKFYQKLRGQFPDAVFWQEIGEIFRQLQKQAAEIYNQSLIELYYEIFIKGKGFANASSVEHYLSDVCYTRAAELFKNAAIASGLRGKVKSNFRLKELKNMKSGLPTTKSDNFPIPLVKQKGGQYTGFEISNLNGDFIIKIPFGRWQVKKEISKYRPWEKFDFEQVRKSPKPISLLLSTQRRKRNKGWSKDEGTEAEIRKVMNGDYQTSYIEVKRGSKIGEKSAWMLNLSIDVPKIDKGVDPSIIGGIDVGVRSPLVCAINNALSRYSISDNDLFHFNKKMFARRRILLKKNRHKRAGHGARNKLKPITILTEKSVRFRKKLIERWACEIADFFIKNKVGTVQMENLESMKRKEDSYFNIRLRGFWPYAEMQNKIEFKLKQYGIEIRRVAPNNTSRTCSKCGHLNSYFNFEYRRKNKFPHFKCEKCNFKEDADYNAALNISNPKLKSTRGEP

SEQ ID NO: 1777 - protein, 726 aa, synthetic construct
SEVEFSHEYWMRHALTLAKRARDEREVPVGAILVLNNRVIGVGWNRAIGLHDPTAHAEIMALRQGGLVMQNYRLIDATLYVTFEPCVMCAGAMIHSRIGRVVFGVRNSKHGAAGSLVNVLNYPGMNHRVEITEGILADECAALLCDFYRMPRQVFNARKKAQSSINSGGSSGGSSGSETPGTSESATPKSSGGSSGGSAKNTITKALKLRIVRPYNSAEVEKIVADEKNNRERIALEKNKDKVKEACSKHLKVAAYCTTQVERNACLFCKARKLDDKFYQKLRGQFPDAVFWQEIGEIFRQLQKQAAEIYNQSLIELYYEILIKGKGFANASSVEHYLSDVCYTRAAELFKNAALASGLRGKVKSNFRLKELKNMKSGLPTTKSDNFPIPLVKQKGGQYTGFEISNHNSDFIIKIPFGRWQAKKEIDKYRPWEKFDFEQVRKSPKPISLLLSTQRRKRNKGWSKDEGTEAEIRKVMNGDYQTSYIEVKRGSKIGEKSAWMLNLSIDVPKIDKGVDPSIIGGIDVGVKSPLVCAINSALSRYSISDNDLFHFNKKMFARRRILLRKNRHKRAGHGAKNKLKPITIMTEKSKRFRKKLIERWACEIADFFIKNKVGTVQMENLESMKRREDSYFNIRLRGFWPYAEMQSRIEFKLRQYGIKIRKVAPNNTSKTCSKCGHLNNYFNFEFRKKNKFPHFKCEKCSFKEDADYNAALNISNPKLKSTKEEP

SEQ ID NO: 1778 - protein, 726 aa, synthetic construct
SEVEFSHEYWMRRALTLAKRARDEREVPVGAVLVLNNRVIGVGWNRAVGLHDPTAHAEIMALRQGGLVMQNYRLIEATLYVTFEPCIMCAGAMIHSRIGRVVFGVRNSKRGAAGSLMNVLNYPGMNHRVEITEGILADECAALISDYYRMPRQVFNARKKAQSSINSGGSSDGGSGSETPGTSESATPESSGGSSGGSAKNTITKTLRLRIVRPFNSAEVEKIVADEKNNREKIALEKNKDKVKEACSEHLKVAAYCTTQVERSACLFCKARKLDDKFYQKLRGQFPDAVFWQEIGEIFRQLQKQAAEIYNQSLIELYYEIFIKGKGFANASSVEHYLSDVCYTRAAELFKNAAIASGLRGKVKSNFRLKELKNMKSGLPTTKSDNFPIPLVKQKGGQYTGFEISNHNSDFIIKIPFGRWQAKKEIDKYRPWEKFDFEQVRKSPKPISLLLSTQRRKRNRGWSKDEGTEAEVKKVMNGDYQISYIEVKRGSKIGERSAWMLNLSIDVPKIDKGVDPSIIGGIDVGVKSPLVCAINNAFSRYSISDNDLFHFNKKMFARRRILLKKSKHKRAGHGAKNKLKPITILTEKSGRFRKKLIERWACEIADFFVKNKVGTVQMENLESMKRKEDSYFNIRLRGFWPYAEMQSKIEFKLKQYGIEIRKVAPNNTSRTCSKCGHLNNYFNFEYRKKNKFPHFKCEKCNFKEDADYNAALNISNPKLKCTKEEP

SEQ ID NO: 1779 - protein, 726 aa, synthetic construct
SEVGFSHEYWMRHALTLAKRARDEREVPVGAVLVLNNRVIGEGWNRAIGLHDPTAHAEIMALRQGGLVMQNYRLIDATLYVTFEPCVMCAGAMIHSRIGRVVFGVRNNKHGAAGSLVNVLNYPGMNHRVEITEGILANECAALLCDFYRMPRQVFNARKKAQSSINPGGSSGGSSSSETPGTSESATPESSGGSSGGSAKNTITKTLKLRIVRPYNSAEVEKIVADEKNNREKIALEKNKDKVKEACSKHLKVAAYCTTQVERNACLFCKARRLDDKFYQKLRGQFPDAVFWQEIGEIFRQLQKQAAEIYNQSLVELYYEILIKGKGIANASSVEHYLSDVCYTRAAELFKNAAIASGLRNKIKSNFRLKELRNMKGGLPTTKSDNFPIPLVKQKGGQYTGFEISSHNSDFIIKIPFGRWQEKEEIDKYRPWEKFDFEQVRRSPKPISLLLSTQRRKKNKGWSKDEGTEAEIRRVMNGDYQTSYIEVKRGSKIGEKSAWMLNLSIDVPKIDKGVDPSIIGGIDVGVKSPLVCAINNAFSRYSISDNDLFHFNKKMFARRRILLKKNRRRRAGHGAKNKLKPITILTEKSVRFRKKLIERWACEIADFFIKNKVGTVQMENLESMKRKEDSYFNIRLRGFWPYAEMQNKIEFKLKQYGIEIRRVAPNNTSRTCSKCGHLNNYFNFEYRRKYKFPHFKCEKCNFKEDADYNAALNISNPKLKSTKEEP

SEQ ID NO: 1780 - protein, 726 aa, synthetic construct
SEVEFSHEYWMRHALTLAKRARDEREVPVGAILVLNNRVIGEGWNRAIGLHDPTAHAEIMALRQGGLVMQNYRLIDATLYVTFEPCVMCAGAMIHSRIGRVVFGVRNSKHGAAGSLVNVLNYPGMNHRVEITEGILADECAALLCNFYRMPRQVFNVRKKAQSSINPGGSSGGSSGSETPGTSESATPESSGGSSASSTKNTITKTLKLRIVRPYNSAEVEKIVADEKNNRERIALEKNKDKVKEACSKHLKMASYCTTQVERNACLFCKARKLDDKFYQKLRGQFPDAVFWQELGGIFRQLQKQAAEIYNQSLIELYYEIFIKGRGFANASSVEHYLSDVCYTRAAELFKNAAIASGLRGKVKSNFRLKELKNMKSGLPTTKSDNFPIPLVKQKGGQYTGFEISSHNDDFVVKIPFGRWQVKKEIDKYRPWERFDFEQVRKSPKPISLLLSTQRRKRNKGWSKDEGTEAEIRKVMNGDYQTSYIEVKRGSKTGEKSAWVLNLSIDVPKIDKGVDPSIIGGIDVGVKSPLVCAINNAFSRYSISDNDLFRFNKKMFARRRILLKKNRHKRAGHGAKNKLKPISILTGKSERFRKKLIERWACEIADFFIKNKVGTVQMENLESMKRKEDSYFNIRLRGFWPYAEMQNKIEFKLKQYGIEIRKVAPNNTSKTCSECGHLNSYFNFEYRKKNKFPHFKCEKCNFKENADYNAALNISNPKLKSTKEEP

SEQ ID NO: 1781 - protein, 726 aa, synthetic construct
SEIEFSHEYWMRHALTLARRARDGREVPVGAVLVLNNRVIGEGWNRAIGLHDPTAHAEIMALRQGGLVTQNYRLIDATLYVTFEPCVMCAGAMVHSRIGRVVFGVRNSKRGAAGSLMNVLDHPGMDHRVEITEGILADECAALLCDFYRMPRQVFNAQKKAQSSINSGGSSGGSSGSETPGTSESATPESSGGSSGGSAKNTITKTLQLRIVRPYNSAEVEKIVTDEKNNREKIALEKNKDKVKEACSKHLKMASYCTTQVERNACLFCKARKLDDKFYQKLRGQFPDAVFWQELGGIFRQLQKQAAEIYNQSLIELYYEILIKGKGVANASSVEHYLSDVCYTRAAELFKNAAIASGLRNKIKSNFRLKELRNMKSGLPTTKSDNFPIPLVRQKGGQYTGFEISNYNGDFIIKIPFGRWQVKKEINKHRPWEKFDFEQVRKSPKPISLLLSTQRRKRNKGWSKDEGTEAEIRKVMNGGYQTSYIEVKRGSKTGEKSAWMLNLSIDVPKIDKGVDPSIIGGIDVGVKSPLVCAINNAFSRYSISDNDLFRFNKKMFARRRILLKKNRHKRAGHGAKNKLKPFTILTEKSGRFRKKLIERWACEIADFFVKNKVGTVQMENLESMKRKEDSYFNIRLRGFWPYAEMQNRIEFKLKQYGIKVRKVAPNNTSKTCSKCGHLNSYFSFEYRKKNKFPHFKCEKCNFKENADYNAALNISNPKMKSTKEEP

SEQ ID NO: 1782 - protein, 726 aa, synthetic construct
SEVEFSHEYWMRHALTLAKRARDEREVPVGAVLVLNNRVIGEGWNRAIGLHDPTAHAEIMALRQGGLVMQNYRLVDATLYVTFEPCVLCAGAMVHSRIGRVVFGVRNSKRGAAGSLMNVLNYPGMNHRVEITEGILADECAALLCDFYRMPRQVFNARKKARSNINSGGSSGGSSGSETPSTSESATPESSGGSSGGSAKNTITKTLTLRIVRPYNSAEVEKIVADEKNNREKIALEKNKDKVKEACSKHLKVAAYCTTQVERNACLFCKARRLDDKFYQKLRGQFPDAVFWQEIGEIFRQLQKQAAEIYNQSLIELYYEIFIKGKGIANASSVEHYLSDVCYTRAAELFKNAAIASGLRNKVKSNFRLKELRSMKSGLPTTKSDNFPIPLVRQKGGQYTGFEISNHNSDFIIKIPFGRWQAKKEIDKYRPWEKFDFEQVRKSPKPISLLLSTQRRKRNRGWSKDESTEAEIKKVMNGDYQTSYIEVKRGSKVGEKSAWMLNLSIDVPKIDKGVDPSIIGGIDVGVKSPLVCAINNVLSRYSISDNDLFHFNKKMFARRRILLKKNGHKRAGHGAENKLKPITIMTEKSKRFRKKLIERWACEIADFFIKNKVGTVQMENLESMKRKEDSYFNIRLRGFWPYAEMQNKIEFKLKQYGIVVRKVAPNNTSKTCSQCGHLNNYFNFEYRKKNQFPYFKCEKCNFKENADYNAALNISNPQLKSTKGEP

SEQ ID NO: 1783 - protein, 726 aa, synthetic construct
SEVEFSHEYWMRHALTLAKRARDEREVPVGAVLVLNNRVIGEGWNRTTGLHDPTAHAEIMALRQGGLVMQNHRLVNATLYVTFEPCVMCAGAMIHSRIGRVVFGVRNSKRGAAGSLTNVLNYPGMNHRVEMTEGILADECAALLCDFYRMPRQVFNGRKKAQSSINSGGSSGGSSGSETPGTSESATPESSGGSSSGSTKNTITKTLKLRIVRPYNSTEVEKIVADEKNNREKIALEKNKDKVKEACSRHLKVAAYCTTQVERNACLFCKARKLDDRFYRKLRGQFPDAVFWQEIGEIFRQLQRQAAEIYNQSLIELYYEIFIKGKGFANASSVEHYLSDVCYTRAAELFKNAAIASGLRGKVKSNFRLKELKNMKSGLPTTKSDNFPIPLVKQKGGQYTGFEISSHNDDFIIKIPFGRWQVKKEIDKYRPWEKFDFEQVRKSPKPISLLLSTQRRKRNKGWSKDEGTEAEIRRVMNGDYQTSYIEVKRGSKIGEKSAWMLNLSIDVPKIDKGVDPSIIGGIDVGVKSPLVCAINNAFRRYSISDNDLFHFNKKMFARRRILLKKNRHKRAGHGVKNKLKPITILTEKSGRFRKKLIERWACEIADFFVKNKVGTVQMENLESMKRKEDSYFNIRLRGFWPYAEMQNKIEFKLKQYGIKVRKVAPNNTSKTCSKCGHLNNYFSFEYRKKNKFPHFKCEKCNFKENADYNAALNISNPKLKSTKEEP

SEQ ID NO: 1784 - protein, 726 aa, synthetic construct
SEDEFSHEYWMRHALTLAKRARDGREVPVGAVLVLNNRVIGEGWNRAIGLHDPTAHAEIMALRQGGLVMQNYRLIDATLYVTFEPCVMCAGAMVHSRIGRVVFGVRNSKRGAAGSLMNVLDYPGMGHRVEITEGILADECAALLCDFYCMPRQVFNAQKRAQSSINSGGSSGGSSGSETPGTSESAIPGSSGGGSSGSAKNTITKTLQLRIVRPYNSAEVEKIVADEKNNREKIALEKNKDKVKEACSEHLKVAAYCTTQVERSACLFCKARKLDDKFYQKLRGQFPDAVFWQEIGEIFRQLQKQAAEIYNQSLIELYYEIFIKGKGFANASSVEHYLSDVCYTRAAELFKNAAIASGLRGKVKSNFRLKELKNMKSGLPTTKSDNFPIPLVKQKGGQYTGFEISNHNSDFIIKIPFGRWQAKKEIDKYRPWEKFDFEQVRKSPKPISLLLSTQRRKKNRGWSKDEGTEAEIRKVMNGDYQTSYIEVKRGSKIGEKSAWMLNLSIDVPKIDKGVDPRIVGGIDVGVKSPLVCAINNAFSRYSISDNDLFHFNKKVFARRRILLKKNRHRRAGHGAKNKLKPISILTEKSKRFRKKLIERWACEIADFFIKNKVGTVQMENLESMKRKEDSYFNIRLRGFWPYAEMQNKIEFKLKQYGIEVRKVAPNNTSKTCSKCGHLNNYFSFEYRKKNKFPHFKCEKCNFKENADYNAALNISNPKLKSTKEEP

SEQ ID NO: 1785 - protein, 726 aa, synthetic construct
SEVEFSHEYWMRHALTLAKRARDGREVPVGAVLVLNNRVIGEGWNRAIGLHDPTAHAEIMALRQGGLVTQNYRLIDATLYVTFEPCAMCAGAMVHSRIGRVVFGVRNSKRGAAGSLMNVLNYPGMGHRVEITEGILADECAALLCDFYCMPRRVFNAQKRAQSSINSGGSSGGGSGSETPGTSESATPESSGGSSGGSAKNTITKTLKLRIVRPFNSAEVEKIVADEKNNREKIALEKNKDKVKEACSEHLKVAAYCTTQVERSACLFCKARKLDDKFYQKLRGQFPDAVFWQEIGEIFRQLQKQAAEIYNQSLIELYYEIFIKGKGFANASSVEHYLSDVCYTRAAELFKNAAIASGLRGKVKSNFRLKELKNMKSGLPTTKSDNFPIPLVKQKGGQYTGFEISNHNDDFIIKIPFGRWQVKKEIDKYRPWEKFDFEQVRKSPKPISLLLSTQRRKRNKGWSKDEGTEAEIRKVMNGDYQTSYIEVRRGSKTGEKSAWMLNLSIDVPKIDKGVDPSIIGGIDVGVRSPLVCAINNAFSRYSISDNDLFHFNKKMFARRRILLKKNRHKRAGHGAKNKLRPISILTEKSGRFRKKLIERWACEIADFFVKNKVGTVQMENLESMKRKEDSYFNIRLRGFWPYAEMQNKIEFKLKQYGIKVRKVAPNNTSKTCSKCGHLNNYFSFEYRKKNKFPHFKCEKCNFKEDADYNAALNISNPKLKNTKGEP

SEQ ID NO: 1786 - protein, 726 aa, synthetic construct
SEVEFSHEYWMRHALTLAKRARDEREVPVGAILVLNNRVIGEGWNRAIGLHDPTAHAEIMALRQGGLVTQNYRLIDATLYVTFEPCVMCAGAMIHSRIGRVVFGVRNSKHGAAGSLVNVLNYPGMNHRVEITEGILADECAALLCDFYRMPRQVFNARKKAQSSINSGGSSGGSSGSETPGTSESATPKSSGGSSSGSAKNTITKTLQLRIVRPYNSAEVEKIVADEKNNREKIALEKNKDKVREACSKHLKVASYCTTQVERNACPFCKARKLDDKFYQKLGGQFPDAVFWQELGEILRQLQKQAAEIYNQSLIELYYEIFIKGRGFANAGSVEHYLSDVCYTRAAELFKNAAIASGLRGKVKSNFRLKELKNMKSGLPTTKSDNFPIPLVKQKGGQYTGFEISSHNDDFIIKIPFGRWQAKKEIDKYRPWEKFDFEQVRKSPKPISLLLSTQRRKRNKGWSKDEGTEAEIRKVMNGDYQTSYIEVKRGSKIGEKSAWMLNLSIDVPKIDKGVDPSIIGGIDVGVKSPLVCAINNAFSRYSISDNDLFHFNKKMFARRRILLKKNRHKRAGHGAKNKLKPISILTGKSERFRKKLIERWACEIADFFVKNKVGTVQMENLESMKGKEDSYFNIRLRGFWPYAEMQNKIEFKLKQYGIKVRKVAPNNTSKTCSKCGHLNNYFSFEYRKKNKFPHFKCEKCNFKENADYNAALNISNPKLKSTKEEP

SEQ ID NO: 1787 - protein, 726 aa, synthetic construct
GEVEFSHEYWMRHALTLAKRARDEREVPVGAALVLNNRIIGEGWNRAIGLHDPTAHAEIMALRQGGLVMQSYRLTDATLYVTFEPCVMCAGAMIHSRIGRVVFGVRNSKRGAAGSLMNVLNYPGMNHRVEITEGILADECAALLCDYYRMPRQVFNARKKAQSSINSGGSSDGGSGSETPGTSESATPESSGGSSGGSAKNTITKTLKLRIVRPYNSAEVEKIVADEKSNREKIALEKNKDKVKEACSEHLKVAAYCTTQVERSACLFCKARKLDDKFYQRLRGQFPDAVFWQELGEIFRQLQKQAAEIYNQSLIELYYEIFIKGKGFANASSVEHYLSDVCYTRAAELFKNAAIASGLRGKVKSNFRLKELKNMKSGLPTTKSDNFPIPLVKQKGGQYTGFEISSHNDDFIIKIPFGRWQVKKEIDKYRPWEKFDFEQVRKSPKPISLLLSTRRRKRNKGWSKDEGTEAEIRKVMNGDYQTSYIEVKRGSKIGEKSAWMLNLSIDVPKIDKGVDPSIIGGIDVGVKSPLVCAINNALSRYSISDNDLFHFNKKMFARRRILLRKNRHKRAGHGAKNKLKPISILTGKSERFRKKLIERWACEIADFFIKNKVGTVQMENLESMKRREDSYFNIRLRGFWPYAEMQNKIEFKLKQYGIEIRKVAPNNTSKTCSKCGHLNNYFNFEYRKKSKFPHFKCEKCNFKENADYNAALNISNPKLKGTKEEP

SEQ ID NO: 1788 - protein, 726 aa, synthetic construct
SEVEFSHEYWMRHALTLAKRARDEREVPVGAVLVLNNRVIGEGWNRAIGLHDPTAHAEIMALRQGGLVMQNYRLTDATLYVTFEPCVMCAGAMIHSRIGRVVFGVRNSKRGAAGSLMNVLNYPGMNHCVEITEGILVDECAALLCDFYRMPRQVLNAQKKAQSSISSGGSSGGSSGSVTPGASGSVTPKSSGGSSAGSTKDTITKTLKLRIVRPYNSAEVEKIVADEKNNREKIALEKNKDKVKEACSKHLEVASYCTTQVERNACPFCKARKLDDKFYQKLRGQFPDAVFWQELGEILRQLQKQAAEIYNQSLIELYYEIFIKGRGFANASSVEHYLSDVCYTRAAELFKNAAIASGLRGKVKSNFRLKELKNMKSSLPTTKSDNFPIPLVKQKGGQYTGFEISSHNDDFIIKIPFGRWQVKKEIDKYRPWEKFDFEQVRKSPKPISLLLSTQRRKRNKGWSKDEGTEAEVRKVMNGDYQTSYIEVKRGSKIGEKSAWMLNLSINVPKIDKGVDPGIIGGIDVGVKSPLVCAVNNALSRYSISDNDLFHFNKKMFARRRILLRKNRHKRAGHGARNKLRPITVLTEKSERFRKKLIERWACEIANFFIKNKVGTVQMENLESMKRREDSYFNIRLRGFWPYAEMQNKIEFKLKQFGIEIRKVAPHNTSKTCSKCGHLNSYFNFEFRKKNKFPHFKCEKCSFKENADYNAALNISNPKLKSTKEEP

SEQ ID NO: 1789 - protein, 726 aa, synthetic construct; identical to SEQ ID NO: 501

SEQ ID NO: 1790 - protein, 726 aa, synthetic construct
SEVEFSHEYWMRHALTLAKRARDEREVPVGAILVLDNRVIGEGWNRAIGLHDPTAHAEIMALRQGGLVMQNYRLTDATLYATFEPCVMCAGAMIHSRIGRVVFGVRNSKHGAAGSLVNVLNYPGMNHRVEITEGILADECAALLCDFYRMPRQVFNARKKAQSSINPGGSSGGSSGSETPGTSESATPESSGGSSGSSAKNTITKTLKLRIVRPYNSAEVEKIVADEKNNREKIALEKNKDKVKEACSKHLKVAAYCTTQVERNACLFCKARRLDDKFYQKLRGQFPDAVFWQEIGEIFRQLQKQAAEVYNQSLVELYYEILIKGKGIANASSVEHYLSDVCYTRAAELFKNAAIASGLRNKIKSNFRLKELRNMKSGLPTTKSDNFPIPLVRQKGGQYTGFEISNHDGDFIIKIPFGRWQVKKEINKHRPWEKFDFEQVRKSPKPISLLLSTQRRKRNRGWSEDEGTEAEIRKVMNGDYQTSYIEVKRGSKIGEKSAWMLNLSIDVPQIDKGVDPSIIGGIDVGVKSPLVCAINNAFSRYSISDNDLFRFNKKMFARRRILLGKNRHKRAGHGVKNKLKPITILTEKSGRFRKKLMERWACEIADFFVKNKVGTVQMENLESMKRKEDSYFNIRLRGFWPYAEMQNKIEFKLKQYGIKVRKVAPNNTSKTCSKCGHLNNYFSFEYRKKNKFPHFKCEKCNFKENADYNAALNISNPKLRSTKEEP

SEQ ID NO: 1791 - protein, 726 aa, synthetic construct
SEVEFSHEYWMRHALTLAKRARDEREVPVGAVLVLNNRVIGEGWNRTIGLHDPTAHAEIMALRQGGLVMQNYRLTDATLYVTFEPCVMCAGAMIHGRIGRVVFGVRNSKRGAAGSLMNVLNYPGMNHCVEITEGILVDECAALLCDFYRMPRQVLNAQKKAQSSISSGGSSGGSSGGETPGASGSVTPKSSGGSSAGSTKDTITKTLKLRIVRPYNSAEVEKIVADEKNNREKIALEKNKDKVKEACSEHLKVAAYCTTQVERNACLFCKARKLDDGFYQKLRGQFPDAVFWQEIGEIFRQLQKQAAEIYNQSLIELYYEIFIKGKGFANASSVEHYLSNVCYTRAAELFKNAAIASGLRGKVKSNFRLKELKNMKSGLPTTKSDNFPIPLVKQKGGQYTGFEISSHNDDLIVKIPFGRWQVKKEIDRHRPWEKFDFEQVRKSPKPISLLLSTQRRKRNKGWSKDEGTEAEIRKVMNGDYQTSYIEVKRGSKIGEKNAWMLNLSIDVPKINKGVDPSIIGGIDVGVKSPLICAINNAFSRYSISDNDLFRFNKKMFARRRILLKKNRHKRAGHGAKNKLKPISILTEKSKRFRKKLIERWACEVADFFIKNKVGTVQMENLESIKRKEDSYFNIRLRGFWPYAEMQNKIEFKLKQYGIEIRKVAPNNTSKTCSKCGHLNNYFNFEYRKKNKFPHFKCEKCNFKENADYNAALNISNPKLKSTKEEP

SEQ ID NO: 1792 - protein, 726 aa, synthetic construct
SEVEFSHEYWMRHALTLAKRARDEREVPVGAVLVLNNRVIGEGWNRTTGLHDPTAHAEIMALRQGGLVMQNHRLVDATLYVTFEPCVMCAGAMIHSRIGRVVFGVRNSKRGAAGSLTNVLNYPGMNHRVEITEGILVGECAGLLCDFYRMPRQVFSARKKAQSSINPGGSSGDSSGGKAPGTSESATLESSGVSSGGSAKSTITKTLKLRIVRPYNSAEVEKIVADEKNNREKTALEKNKGKVKEACSKHLKVATYCTTQVERNACLFCKARKLDDKFYQKLRGQFPDAVFWQEIGEIFRQLQKQAAEIYNQSLIELYYEIFIKGKGFANASSVEHYLSDVCYTRAAELFKNAAIASGLRGKVKSNFRLKELKNMKSGLPTTKSDNFPIPLVKQKGGQYTGFEISSHNDDFIIKIPFGRWQVKKEIDRYRPWEKFDFEQVRKSPKPISLLLSTQRRKRNKGWSKDEGTEAEIRKVMNGDYQTSYIEVKRGSKIGEKSAWMLNLSIDVPKIDKGADPSIIGGIDVGVKSPLVCAINNAFSRYSISDNDLFHFNKKMFARRRILLKKNRHKRAGHGAKNKLKPITILTEKSGRFRKKLIERWACEIADFFIKNKVGTVQMENLGSMKRKEDSYFNIRLRGFWPYAEMQNKIELKLKQYGIKIRKVAPNNTSKTCSKCGHLNDYFNFEYRKKNKFPHFKCEKCNFKEDADYNAALNISNPKLKGTREEP

SEQ ID NO: 1793 - protein, 726 aa, synthetic construct
SEVEFSHEYWMRHALTLAKRARDEREVPVGAILVLNNRVIGEGWNRAIGMHDPTAHAEIMALRQGGLVMQNYRLVDATLYVTFEPCVLCAGAMVHSRIGRVVFGVRNSKRGAAGSLMNVLNYPGMNHRVEVTEGILADECAALLCDFYRMPRQVFNARKKARSNINPGGSSGGSSGGKAPGTSESATLESSGGSSGGSAKNSITKTLKLRIVRPYNSAEVEKIVADEKNNREKIALEKNKGKVKEACSKHLKVATYCTTQVERNACLFCRARKLDDKFYQKLRGQFPDAVFWQELGGIFRQLQKQAAEIYNQSLIELYYEIFIKGKGITNASRVEHYLSDVCYTRAAELFKNAAIASGLRSKVRSNFRLKELKNMKSGLPTTKSDNFPIPLVKQKGGQYTGFEISSHNDDFIIKIPFGRWQAKKEIDKYRPWEKFDFEQVRKSPKPISLLLSTQRRKRNKGWSKDEGTEAEIRKVMNGDYQTSYIEVKRGSKIGEKSAWMLNLSIDVPKIDKGVDPSIIGGIDVGVKSPLVCAINNAFSRYSISDNDLFRFNKKMFARRRILLKKNRHKRAGHGAKNKLKPITILTEKSVRFRKKLIERWACEIADFFVKNKVGTVQMENLESMKRKEDSYFNIRLRGFWPYAEMQNKIEFKLKQYGIVVRKVAPNNTSKTCSQCGHLNNYFNFEYRKKNKFPHFKCERCNFKENADYNAALNISNPKLKSTKEES

SEQ ID NO: 1794 - protein, 726 aa, synthetic construct
SEVEFSHEYWMRHALTLAKRARDEREVPVGAVLVLNNRVIGEGWNRAIGLHDPTAHAEIMALHQGGLVMQNYRLIDATLYVTFEPCVMCAGAMIHSRIGRVVFGARNSKRGAAGSLMNVLSYPGMNHRVEITEGILVDECAALLCDFYRMPRQVLSAQKKAQSSVSSGGSSGGSSGSETPGASGSVTPKGSGGSSAGSTKDTITKTLKLRIVRPYNSAEVEKVVADEKNNREKIAMEKNKDKVKEACSKHLKVASYCTTQVERNACLFCKARKLDDKFYQKLRGQFPDAVFWQELGGIFRQLQKQAAEIYNQSLIELYYEIFIKGKGFANASSVEHYLSDVCYTRAAELFKNAAIASGLRGKVKSNFRLKELKNMKSGLPTTKSDNFPIPLVKQKGGQYTGFEISSHDDDFIIKIPFGRWQVKEEIDKYRPWEKFDFEQVRKNPKPISLLLSTQRRKRNKGWSKDEGTEAEIRKVMNGDYQTSYIEVKRGSKTGEKSAWMLNLSIDVPKIDKGVDPSIIGGIDVGVKSPLVCAINNALSRYSISDNDLFHFNKKIFARRRILLKKNRHKRAGHGAKNKLKPITILTEKSVRFRKKLIERWACEIADFFIKNKVGTVQMENLESMKRKEDSYFNIKLRGFWPYAEMQNKIEFKLKQYGIEIRKVAPDNTSKTCSKCGHLNNYFNFEYRKKNKFPHFKCEKCNFKEDADYNAALNISNPKLKSTKEEP

SEQ ID NO: 1795 - protein, 726 aa, synthetic construct
SEVEFSHEYWMRHALTLAKRARDEHEVPVGAVLVLNNRVIGEGWNRAIGLHDPTAHAEIMALRQGGLVLQNYRLVDATLYVTFEPCVLCAGAMVHSRIGRVVFGARNSKRGAAGSLMNILNYPGMNHHVEITEGILVDECAALLCDFYRMPRQVFNAQKKAQSTINSGGSSGGSSGSETPGTSESPTPESSGGSPGGSAKNTITKTLKLRIVRPYNSAEVEKIVADEKNNREKIALEKNKDKVKEACSKHLKVAAYCTTQVERNACLFCKARKLDDKFYQKLRGQFPDAVFWQEIGEIFRQLQKQAAEIYNQCLIELYYEIFIKGKGFANASSVEHYLSDVCYTRAAELFKNAAIASGLRGKVKSNFRLKELKNMKSGLPTTKSDNFPIPLVKQKGGQYTGFEISSHNDDFIIKIPFGRWQVKEEIDKYRPWEKFDFEQVRKNPKPISLLLSTQRRKRNKGWSKDEGTEAEIRKVMNGDYQTSYIEVKRGSKIGEKSAWMLNLSIDVPKIDKGVDPSIIGGIDVGVKSPLVCAINNAFSRYSISDNDLFHYNKKMFARRRILLKKNRHKRAGHGAKNKLKPITILSEKSKRFRKKLIERWACEIADFFIKNKVGTVQMENLESMKRKEDSYFNIRLRGFWPYAEMQNKIEFKLKQYGIEIRKVAPNNTSRTCSKCGHLNNYFSFEYRKKNKFPHFRCEKCNFKEDADYNAALNISNPKLKSTKEEP

SEQ ID NO: 1796 - protein, 726 aa, synthetic construct
SEDEFSHEYWMRHALTLAKRARDGREVPVGAVLVLNNRVIGEGWNRAIGLHDPTAHAEIMALRQGGLVMQNYRLIDATLYVTFEPCVMCAGAMVHSRIGRVVFGVRNSKRGAAGSLMNVLDYPGMGHRVEITEGILADECAALLCDFYCMPRQVFNAQKRAQSSINSGGSSGGSSGSDTQGTSESATPESSGGSSSGSVKNTITKTLQLRIVRPYNSAEVEKIVADEKNNREKIALEKNKDKVKEACSKHLKVASYCTTQVERNACPFCKARKLDDKFYQKLRGQFPDAVFWQEIGEIFRQLQKQAAEIYNQSLVELYYEILIKGKGFANASSVEHYLSDVCYTRAAELFKNAAIASGLRGKVKGNFRLKELKNMRSGLPTTKSDNFPIPLVKQKGGQYTGFEISSHNDDFIIKIPFGRWQAKKEIDKYRPWEKFDFEQVRKSPKPISLLLSTQRRKRNKGWSKNEGTEAEIRKVMNGDYQTSYIEVKRGSKIGEKSAWMLNLSIDVPKIDKGVDPSIIGGIDVGVKSPLVCAINNAFSRYSISDNDLFHFNKKMFARRRILLKKNRHKRAGHGAKNKLKPISTLTGKSKRFRKKLIERWACEIADFFIKNKVGTVQMENLESMKRKGDSYFNIRLRGFWPYAEMQNKIEFKLKQYGIEIRKVAPNNTSKTCSKCGHLNNYFNFEYRRKNKFPHFKCEKCNFKEDADYNAALNISNPKLKSTKEEP

SEQ ID NO: 1797 - protein, 726 aa, synthetic construct
SEVEFSHEYWMRHALTLAKRARDEREVPVGAILVLNNRVIGEGWNRAIGLHDPTAHAEIMALRQGGMVMQNYRLINATLYVTFEPCVMCAGAMIHSRIGRVVFGVRNSKHGAAGSLMNVLNYPGMNHRVEITGGILADECAALLCDFYRMPRQVFNAQKKARSNINSGGSSGGSSGSETLGTSESATPESSGGSSGGSAKNTITKTLKLRIVRPYNSAEVEKIVADEKNNREKIALEKNKDKVKEACSEHLKVAAYCTTQVERNACLFCKARKLDDKFYQKLRGQFPDAVFWQEIGEIFRQLQRQAAEIYNQSLIELYYEIFIKGKGFANASSVEHYLSDVCYTRAAELFKNAAIASGLRGKVKSNFRLKELKNMKSGLPTTKSDNFPIPLVKQKGGQYTGFEISSHNDDFIIKIPFGRWQVKKEIDKYRPWEKFDFEQVRKSPKPINLLLSTQRRKRNKGWSKDEGTEAEIRKVMNGDYQTSYIEVKRGSKIGEKSAWMLNLSIDVPKIDKGVDPSIVGGVDVGVKSPLVCAINNAFSRYSIGDNDLFHYNKKMFARRRILLKKNRHKRAGHGAKNKLKPISILTEKSKRFRKKLIERWACEIADFFIKNKVGTVQMENLESMKRKEDSYFNIRLRGFWPYAEMQNKIEFKLKQYGIEIRKVAPNNTSRTCSRCGHLNNYFNFEYRKENKFPHFKCEKCNFKEDADYNAALNISNPELKSTKEEP

SEQ ID NO: 1798 - protein, 726 aa, synthetic construct; identical to SEQ ID NO: 1621

SEQ ID NO: 1799 - protein, 726 aa, synthetic construct
SEDEFSHEYWMRHALTLAKRARDGREVPVGAVLVLNNRVIGEGWNRAIGLHDPTAHAEIMALRQGGLVMQNYRLTDATLYATFEPCVMCAGAMIHSRIGRVVFGVRNSKHGAAGSLMNVLNYPGMNHRVEITEGILADECAALLCDFYRMPRQVFNARKKARSNINSGGSSGGSSGSETPGTSESATPESSGGSPGGSAKNTITKTLKLRIVRPYNSAEVEKIVADEKNNREKIALEKNKDKVKEACSKHLKVAAYCTTQVGRNACLFCKARKLDDKFYQKLRGQFPDAVFWQEIGEIFRQLQKQAAEIYNQSLIELYYEIFIKGKGFANASSVEHYLSDVCYTRAAELFKNAAIASGLRGKVKSNFRLKELKNMKSGLPTTKSDNFPIPLVKQKGGQYTGFEISSHNDDFIIKIPFGRWQVKEEIDKYRPWEKFDFEQVRKNPKPISLLLSVQRRKRNKGWSRDEGTEAEIRKVMNGDYRTSYIEVKRGSKIGEKSAWMLNLSIDVPKIDKGVDPSIIGGIDVGVKSPLVCAIDNAFSRYSISDNDLYRFNKKMFARRRILLKKNRHKRAGHGAMNKLKPITILTEKSGRFRKKLIERWACEIADFFIKNKVGTVQMENLESMKRREDSYFNIRLRGFWPYAEMQNKIEFKLKQYGIVVRKVAPNNTSKTCSKCGHLNNYFNFEFRKKNKFPHFKCEKCNFKEDADYNAALNISNPKLKSTKEEP

SEQ ID NO: 1800 - protein, 726 aa, synthetic construct
SEVEFSHEYWMRHALTLAKRARDEREVPVGAILVLNNRVIGEGWNRAIGLHDPTAHAEIMALRQGGLVMQNYRLIDATLYVTFEPCVMCAGAMVHSRIGRVVFGVRNSKRGAAGSLMNVLDYPGMGHRVEITEGILADECAALLCDFYCMPRQVFNAQKRAQSSINSGGSSSGSSGSDTPGTSESATPESSGGGSSGSAKNTITKTLQLRIVRPYNSAEVEKIVADEKNNREKIALEKNKDKVREACSKHLKVASYCTTQVERNACPFCKARKLDDKFYQKLRGQFPDAVFWQELGEIFRQLQRQAAEIYNRSLIELYYEIFIKGRGFANASSVEHYLSDVCYTRAAELFKNAAIASGLRGKVKSNFRLKELKNMKSGLPTTKSDNFPIPLVKQKGGQYTGFEISSHNDDFIIKIPFGRWQVKKEIDKYRPWEKFDFEQVRKSPKPISLLLSTQRRKRNKGWSKDEGTEAEIRKVMNGDYRTSYIEVKRGSKTGEKSAWVLNLSIDVPKIDKGVDPSIIGGIDVGVKSPLVCAINNAFSRYSISDNDLFRFNKKMFARRRILLGKNRHKRAGHGVKNKLKPITILTEKSGRFRKKLIERWACEIADFFVKNKVGTVQMENLESMKRKEDSYFNIRLRGFWPYAEMQNKIEFKLKQYGIGIRKVAPNNTSKTCSKCGHLNNYFNFEYRKKNKFPHFKCEKCNFKESADYNAALNISNPKLKSTKEEP

SEQ ID NO: 1801 - protein, 726 aa, synthetic construct
SEVEFSHEYWMRHALTLAKRARDEREVPVGAVLVLNNRVIGEGWNRAIGLHDPTAHAEIMALRQGGLAMQNYRLVDATLYVTFEPCVLCAGAMVHSRIGRVVFGVRNSKRGAAGSLMNVLNHPGMNHRVEITEGILADECAALLCDFYRMPRQVFNARKKAQSNINSGGLSGGNSGSETPGASESPTPESSGSSSGGPAKNTITKTLKLRIVRPYNSAEVEKIVADEKNNREKIALEKNKDKVKEACSKHLKMASYCTTQVERNACLFCKARKLDDKFYQKLRGQFPDAVFWQELGEIFRQLQKQAAEIYNQSLIELYYEIFIKGKGIANASRVEHYLSDVCYTRAAELFKNAAIASGLRSKVRSNFRLKELKNMKSGLPTTKSDNFPIPLVKQKGGQYTGFEVGSHNSDFIIKIPFGRWQVKEEIDKYRPWEKFDFEQVRKSPKPISLLLSTQRRKKNKGWSKDEGTEAEIRRVMNGDYQTSYIEVKRGSKIGEKSAWMLNLSIDVPKIDKGVDPSIIGGIDVGVKSPLVCAINNSLSRYSICDNDLFRFNKKMFARRRILLKKNRHKRAGHGAKNKLKPITILTKKSERFRKKLIERWVCEVADFFIKNKVGTVQMENLESMKRKEDSYFNIRLRGFWPYAEMQNRIELKLKQYGIEIRRVAPNNTSRTCSRCGHLNNYFNFEYRKKSKFPHFKCEKCNFREDADYNAALNISNPKLKSTKEEP

SEQ ID NO: 1802 - protein, 726 aa, synthetic construct
SEDEFSHEYWMRHALTLAKRARDGREVPVGAVLVLNNRVIGEGWNRAIGLHDPTAHAEIMALRQGGLVMQNYRLIDATLYVTFEPCVMCAGAMVHSRIGRVVFGVRNSKRGAAGSLMNVLDYPGMGHRVEITEGILADECAALLCDFYCMPCQVFNAQKRAQSSINSGGSSGSSSGSDTPGTSKSATPESSGGSSGDSAKNTITKTLQLRIVRPYNSAEVEKIVADEKNNREKIALEKNKDKVREACSKHLKVASYCTTQVERNACPFCKARKLDDKFYQKLRGQFPDAVFWQELGEILRQLQKQAAEIYNQSLIELYYEIFIKGRGFANASSVEHYLSDVCYTRAAELFKNAAIASGLRGKVKSNFRLKELKNMKSGLPTTKSDNFPIPLVKQKGGQYTGFEISSHNSDFIIKIPFGRWQVKKEINKYRPWEKFDFEQVRKSPKPISLLLSTQRRKRNKGWSKDEGTEAEIRKVMNGDYQTSYIEVKRGSKIGEKSAWVLNLSIDVPKIDKGVDPSIIGGIDVGVKSPLVCAINNAFSRYSISDNDLFRFNKKVFARRRILLKKNRHKRAGHGTKNKLRPITILAEKSGRFRKKLIERWACEIANFFIKNKVGTVQMENLESMKRKEDSYFNIRLRGFWPYAEMQNKIEFKLKQYGIEIRKVAPNNTSKTCSKCGHLNNYFSFEYRKKNKFPHFKCEKCNFKEDADYNAALNISNPKLKSTKEEP

SEQ ID NO: 1803 - protein, 726 aa, synthetic construct
SEVEFSHEYWMRHALTLAKRARDEREVPVGAVLVLNNRVIGEGWNRAIGLHDPTAHAEIMALRQGGLVMQNYRLVDATLYVTFEPCVLCAGAMVHSRIGRVVFGVRNSKRGAAGSLMNVLNYPGMNHRVEITEGILADECAALLCDFYRMPRQVFNAQKKARSNTNSGGSSGGSSGSETPGTSESATPVSSSGSPGGSAKNTITKTLKLRIVRPYNSAEVEKIVADEKNNREKIALAKNKDKVKEACSEHLKVAAYCTTQVERNACLFCKARKLDDKFYQKLRGQFPDAVFWQEIGEIFRQLQKQAAEIYNQSLIELYYEIFIKGKGFANASSVEHYLSDVCYTRAAELFKNAAIASGLRGKVKSNFRLKELKNMKSGLPTTKSDNFPIPLVRQKGGQYTGFEISNHDGDFTIKIPFGRWQVKKEINKHRPWEKFDFEQVRKSPKPISLLLSTQRRKRNKGWSKDEGTEAEIRKVMNGDYQTSYIEVKRGSKIGEKSAWMLNLSIDVPKIDKGVDPSIIGGIDVGVKSPLVCAINNALSRYSISDNDLFHFNKKMFARRRILLRKNRHKRAGHGAKNKLKPITTMTEKSKRFRKKLIERWACEIADFFIKNKVGTVQMENLESMKRKEDSYFNIRLRGFWPYAEMQSKIEFKLKQYGIVVRKVAPNNTSKTCSKCGHLNNYFNFEYRKKNKFPHFKCEKCNFKEDADYNAALNISNPKLKSTKGEP

SEQ ID NO: 1804 - protein, 726 aa, synthetic construct; identical to SEQ ID NO: 684

SEQ ID NO: 1805 - protein, 726 aa, synthetic construct
SEVEFSHEYWMRHALTLAKRARDEREVPVGAILVLNDRVIGVGWNRAIGLHDPTAHAEIMALRQGGLVMQNYRLIDATLYVTFEPCVMCAGAMIHSRIGRVVFGVRNSKHGAAGSLVNVLNYPGMNHRVEITEGILADECAALLCDFYRMPRQVFNARKKAQSSINSGGSSGGSSGSETPGTNESATPKSSGGSSGGSAKNTITKALKLRIVRPYNSAEVEKIVADEKNNREKIALEKNKDKVREACSEHLKVAAYCTTQVEKNACLFCKARKLDDKFYQRLRGQFPDAVFWQEISEILRQLQKQAAEIYNQSLIELYYEIFIKGKGFANASSVEHYLSDVCYTRAAELFKNAAIASGLRGKVKSNFRLKELKNMKSGLPTTKSDNFPIPLVKQKGGQYTGFEISSHNDDFIIKIPFGRWQVKKEVDKYRPWEKFDFEQVRKSPKPISLLLSTQRRKRNKGWSKDEGTEAEIRKVMNGDYQTSYIEVKRGSKIGEKSAWMLSLSIDVPKIDKGVDPSIIGGIDVGVKSPLVCAINNAFCRYSISDNDLFHFNKKMFARRRILLKKSRHKRAGHGAKNKLKPISILTEKGKRFRKKLIERWASEIADFFIKNRVGTVQMENLESMKRREDSYFNIRLRGFWPYAEMQSKIEFKLKQYGIKIRKVAPNNTSKTCSKCGHLNNYFNFEFRKKNKFPHFKCEKCNFKEDADYNAALNISNPKLKSTKEEP

SEQ ID NO: 1806 - protein, 726 aa, synthetic construct
SEVEFSHEYWMRHALTLAKRARDEREVPVGAVLVLNNRVIGVGWNRAIGLHDPTAHAEIMALRQGGLVMQNYRLIDAALYVTFEPCIMCAGAMIHSRIGRVVFGVRNSKRGAAGSLMNVLNYPGMNHRVEITEGVLADECAALLCDFYRMPRQVLNAQKKAQSSINSGGSSGGGSGGETPGTSESATQESFGGSSGGSAKNTITKTLKLRIVRPYNSAEVEKIVADEKNNREKIALEKNKDKVKEACSKHLKVASYCTTQVERNACLFCKARKLDDKFYQKLRGQFPDAVFWQELGEIFRQLQKQAAEIYNQSLIELYYEIFIKGKGFANASSVEHYLSDVCYTRAAELFKNAAIASGLRGKVKSNFRLKELKNMKSGLPTTKSDNFPIPLVKQKGGQYTGFEISSHNDDFIIKIPFGRWQVKREIDKYRPWEKFDFEQVRRSPKPISLLLSTQRRKKNKGWSKDEGTEAEIRRVMNGDYQTSYIEVKRGSKIGEKSAWMLNLSIDVPKIDKGVDPSIIGGIDVGVKSPLVCAINNAFSRYSISDNDLFRFNKKMFARRRILLKKNRHKRAGHGAKNKLKPISILTGKSERFRKKLIERWACEIADFFIKNKVGTVQMENLESMKRKEDSYFNIRLRGFWPYAEMQNKIEFKLKQYGIEIRKVAPNNTSKTCSKCGHLNNYFNFEYRKKNKFPHFKCEKCNFKESADYNAALNISNPKLKSTKEEP

SEQ ID NO: 1807 - protein, 726 aa, synthetic construct
SEDEFSHEYWMRHALTLAKRARDGREVPVGAVLVLNNRVIGEGWNRAIGLHDPTAHAEIMALRQGGLVMQNYRLIDATLYVTFEPCVMCAGAMIHSRIGRVVFGVRNSKHGAAGSLMNVLNYPGMNHRVEITEGILVDECAALLCDFYRMPRQVFNARKKAQSSINPGGSSGGSSGSEMPGTSESATPGSSGGSSGGSAKNTITKTLKLRIVRPYNSAEVEKIVADEKNNREKIALEKNKDKVREACSKHLKVAAYCTTQVERNACLFCKARKLDDKFYQKLRGQFPDAVFWQEIGEIFRQLQKQAAEIYNQSLIELYYEIFIKGKGITNASRVEHYLSDVCYTRAAELFKNAAIASGLRSKVRSNFRLKELKNMKSGLPTTKSDNFPIPLVKQKGGQYTGFEISSHNSDFIIKIPFGRWQVKEEIDKYRPWEKFDFEQVRKSPKPISLLLSTQRRKKNKGWSKDEGTEAEIRRVMNGDYQTSYIEVKRGSKIGEKSAWMLNLSIDVPKIDKGVDPSIIGGIDVGVKSPLVCAINNAFSRYSISDNDLFHFNKKMFARRRILLKKNRHKRAGHGAKNKLKPLTILTGKSKRFRKKLIERWACEIADFFIKNKVGTVQMENLESMKRKEDSYFNIRLRGFWPYAEMQNKIEFKLKQYGIEIRKVAPSNTSKTCSRCGHLNNYFNFEYRKRNKFPHFKCERCNFKENADYNAALNISNPKLKSPKEEP

SEQ ID NO: 1808 - protein, 726 aa, synthetic construct
SEDEFSHEYWMRHALTLAKRARDGREVPVGAVLVLNNRVIGEGWNRAIGLHDPTAHAEIMALRQGGLVMQNYRLIDATLYVTFEPCVMCAGAMIHSRIGRVVFGVRNSKRGAAGSLMNVLNYPGMNHRVEITEGVLADECAALLCDFYRMPRQVLNAQKKAQSSINSGGSSGGGSGGETPGTSESATQESSGGSSGGSAKNTITKTLKLRIVRPYNSAEVEKIVADEKNNREKIALEKNKDKVKEACSEHLKVAAYCTTQVERSACLFCKARKLDDKFYQKLRGQFPDAVFWQELGEIFRQLQKQAAEIYNQSLIELYYEIFIKGKGLANASSVEHYLSDVCYTRAAELFKNAAIASGLRGKVKSNFKLKELKSMKSGLPSTKSDNFPIPLVKQKGGQYTGFEISSHNDDLIIKIPFGRWQVKREIDKYRPWEKFDFEQVRKSPKPISLLLSTQRRKRNKGWSKDEGTEAEIRKVMNGDYQTSYIEVKRGSKIGEKSAWMLNLSIDVPKIDKGVDPSIIGGIDVGVKSPLVCAINNAFSRYSISDNDLFHFNKKMFARRRILLKKNRHKRAGHGAKNKLKPISILTEKSERFRKKLIERWACEIADFFIKNKVGTVQMENLESMKRREDSYFNTRLRGFWPYAEMQNKIEFKLKQYGIEIRKVAPNNTSKTCSKCGHLNNYFNFEYRKKNKFPHFKCEKCNFKENADYNAALNISNPKLKSTKEEP

SEQ ID NO: 1809 - protein, 726 aa, synthetic construct
SEVEFSHEYWMRRALTLAKRARDEREVPVGAVLVLNNRVIGVGWNRAIGLHDPTAHAEIMALRQGGLVMQNYRLIDATLYVTFEPCVMCAGAMIHSRIGRVVFGVRNNKHGAAGSLVNVLNYPGMNHRVEITGGILADECAALLCDFYRMPRQVFNARKKAQSSINPGGSSGGSSGSETPGTSESATPESSGGSSGGSAKNTITKTLKLRIVRPYNSAEVEKIVADEKNNREKIALEKNKDKVKEACSKHLKVASYCTTQVERNACLFCKARKLDDKFYQKLRGQFPDAVFWQEIGEIFRQLQKQAAEIYNQSLIELYYEIFIKGKGFANASSVEHYLSDVCYTRAAELFKNAAIASGLRGKVKSNFRLKELKNMKSGLPTTKSDNFPIPLVKQKGGQYTGFEISSHNDDFIIKIPFGRWQVKKEIDKYRPWEKFDFEQVRKSPKPISLLLSTQRRKRNKGWSKDEGTEAEIRKVMNGDYQTSYIEVKRGSKIGEKSAWMLNLSIDVPKIDKGVDPSIIGGIDVGVKSPLVCAINNAFSRYSISDNDLFHFNKKMFARRRILLKKNGHKRAGHGAKNKLRPITIMTEKSKRFRKKLIERWACEIADFFIKNKVGTVQMENLEGMKGREDSYFNIRLRGFWPYAEMQNKIEFKLKQYGIEVRKVAPNNTSKTCSKCGHLNNYFNFEYRKKNKFPHFKCEKCNFKENADYNAALNISNPKLKSTKEEP

SEQ ID NO: 1810 - protein, 726 aa, synthetic construct
SEVEFSHEYWMRHALTLAKRARDEREVPVGAILVLNNRVIGVGWNRAIGLHDPTAHAEIMALRQGGLVTQNYRLIDATLYVTFEPCVMCAGAMIHSRIGRVVFGVRNNKHGAAGSLVNVLDYPGMNHRVEITEGILADECAALLCDFYRMPRQVFNARKKAQSSINSGGSSGGSSGSEAPGTSESATPESSGGNSGGSAKNTITKTLKLRIVRPYNSAEVEKIVADEKNNREKIALEKNKDKVKEACSEHLKVAAYCTTQVERNACLFCKARKLDDKFYQKLRGQFPDAVFWQEIGDIFRQLQKQAAEIYNQSLIELYYEIFIKGKGFANASSVEHYLSDVCYTRAAELFKNAAIASGLRGKVKSNFRLKELKNMKSGLPTTKSDNFPIPLVKQKGGQYTGFEISNHNSDFIIKIPFGRWQAKKEIDKYRPWEKFDFEQVRKSPKPISLLLSTQRRKRSKGWSKDEGTEAEIRKVMNGDYQTSYIEVKRGSKIGEKSAWMLNLSIDVPKIDKGVDLSIIGGIDVGVKSPLVCAINNALSRYSISDNDLFHFNKKMFARRRILLRKNRHKRAGHGARNKLKPITVLTEKSERFRKKLIERWACEIANFFIKNKVGTVQMENLESMKRREDSYFNIRLRGFWPYAEMQSKIEFKLKQYGIKIRKVAPNNTSKTCSKCGHLNNYFNFEFRKKNKFPHFKCEKCNFKEDADYNAALNISNPKLKSTKEEP

SEQ ID NO: 1811 - protein, 726 aa, synthetic construct
SEVEFSHEYWMHHALTLAKRARDEREVPVGAILVLNNRVIGEGWNRAIGLHDPTAHAEIMALRQGGLVMQNYRLIDATLYVTFEPCVMCAGAMIHSRIGRVVFGVRNNKHGAAGSLVNVLNYPGMNHRVEITEGILADECAALLCDFYRMPRQVFNARKKAQSSINPGGSSGGSSGSETPGTSESATPESSGGSSGSSAKNTITKTLKLRIVRPYNSAEVEKIVADEKNNREKIALEKNKDKVKEACSKHLKVAAYCTTQVERNACLFCKARKLDDKFYQKLRGQFPDAVFWQELGEIFRQLQKQAAEIYNQSLIELYYEIFIKGKGFANASSVEHYLSDVCYTRAAELFKNAAIASGLRGKVKSNFRLKELKNMKSGLPTTKSDNFPIPLVKQKGGQYTGFEISSHNDDFTIKIPFGRWQVKKEIDKYRPWEKFDFEQVRKSPKPISLLLSTQRRKRNKGWSKDEGTEAEIRKVMNGDYQTSYIEVKRGSRIGEKSAWMLSLSIDVPKIDRGVDPSIIGGIDVGVKSPLVCAIDNALSRYSISDNDLFHFNKKMFARRRVLLKKNRHRRAGHGAKNKLKPISILTEKSKRFRKKLIERWACEIADFFIKNKVGTVQMENLESMKRKEDSYFNIRLRGFWPYAEMQNKIEFKLKQYGIEIRKVAPNNTSKTCSKCGHLNNYFNFEYRKKNKFPHFKCEKCYFKEDADYNAALNISNPKLKSTKEEP

SEQ ID NO: 1812 - protein, 726 aa, synthetic construct; identical to SEQ ID NO: 684

SEQ ID NO: 1813 - protein, 726 aa, synthetic construct
SEVEFSHEYWMRHALTLAKRARDEREVPVGAVLVLDNRVIGEGWNRAIGLHDPTAHAEIMALRQGGLEMQNYRLIDATLYVTFEPCAMCAGAMVHSRIGRVVFGVRNSKRGAAGSLMNVLNYPGMDHRVEITGGILADECAALLCDFYRMPRRVFNAQKKAQSSISSGGSSGGSSGSETPGASGSVTPKSSGGSSAGSTKDTITKTLKLRIVRPYNSAEVEKVVADEKNNREKIAIEKNKDMVKEACSKHLKVASYCTTQVERNACLFCKARKLDDKFYQKLRGQFPDAVFWQELGGIFRQLQKQAAEIYNQSLIELYYEIFIKGKGITNASRVEHYLSDVCYTRAAELFKNAAIASGLRSKVRSNFRLKELRNMKSGLPTTRSDNFPIPLVRQKGGQYTGFGISNHNSDFIIKIPFGRWQVKKEIDKYRPWEKFDFAQVRKSPKPISLLLSTQRRRRNKGWSNDEGTEAEIRKVMNGDYQTSYIEVKRGSKIGEKSAWMLSLSIDVPKIDKGVDPSIVGGIDVGVKSPLVCAINNALGRFSISDNDLFHFNKKMFARRRILLRKNRHKRAGHGAKNKLKPISILTEKSRRFRKKLIERWACEIADFFIKNKVGTVQMEDLESMKRRGDSYFNIRLRGLWPYAEMQNKIEFKLKQYGIEIRKVAPNNTSKTCSKCGHLNNYFNFEYRKKNKFPHFKCEKCNFKENADYNAALNISNPKLKNTKEEP

SEQ ID NO: 1814 - protein, 726 aa, synthetic construct
SEVEFSHEYWMRHALTLAKRARDEREVPVGAILVLNNRVIGEGWNRATGLHDPTAHAEIMALRQGGLVMQNYRLTDATLYVTFEPCVMCAGAMIHSRIGRVVFGVRNNKHGAAGSLVNVLNYPGMNHRVEITEGILANECAALLCDFYRMPRQVFNARKKAQSSINSGGSSGGSSGSETPGTSESATPESSGGGSSGSAKNTITKTLQLRIVRPYNSAEVEKIVADEKNNREKIALEKNRDKVKEACSKHLKVAAYCTTQVERSACLFCKARRLDDKFYQKLRGQFPDAVFWQEISEIFRQLQKQAAVIYNQSLIELYYEIFIKGKGIASASRVGHYLSDVCYTRAAELFKNAAIASGLRSKIKSNFRLKELKNMKSGLPTTKSDNFPIPLVKQKGGQYTGFEISDHNGDFIIKIPFGRWQVKKEIDKYRPWEKFDFEQVRKSPKPISLLLSTRRRKRNKGWSKDEGTEAEIRKVMNGDYQTSYIEVKRGSKIGEKSAWMLNLSIDVPKVDKGVDPSIIGGIDVGVKSPLVCAINNAFSRYSISDNDLFHFNKKMFARRRILLKKNGHKRAGHGARNKLKPITIMTEKSKRFRKKLIERWACEIADFFVKNKVGTVQMENLESMKRKEDSYFNIRLRGFWPYAEMQSKIEFKLKQYGIVVRKVTPNNTSKTCSKCGHLNSYFNFEYRKKNKFPHFKCEKCNFKENADYNAALNICNPKLKSTKEEP

SEQ ID NO: 1815 - protein, 726 aa, synthetic construct
SEVEFSHEYWMRHALTLAKRARDEREVPVGAILVLNNRVIGEGWNRAIGLHDPTAHAEIMALRQGGLVMQNYRLIDATLYVTFEPCVMCAGAMIHSRIGRVVFGVRNNKHGAAGSLVNVLNYPGMNHRVEITEGILADECAALLCDFYRMPRQVFNARKKAQSSINPGGSSGGSSGSETPGTSESATPESSGGSSGSSAKNTITKTLKLRIVRPYNSAEVEKIVADEKNNREKIALEKNKDKVKEACSKHLKVAAYCTTQVERNACLFCKARRLDDKFYQKLRGQFPDAVFWQEIGEIFRQLQKQAAEVYNQSLVELYYEIFIKGKGITNASRVEHYLSDVCYTRAAELFKNAAIASGLRSKVRSNFRLKELKNMKSGLPTTKSDNFPIPLVKQKGGQYTGFEISSHNDDFIIKIPFGRWQVRKEIDKYRPWEKFNFEQVRKSPRPISLLLSTQRRKRNKGWSKDEGTEAEIRKVMNGDYQTSYIEVKRGSKIGEKSAWMLSLSIDVPKIDKGVDPSIIGGIDVGVKSPLVCAINNAFNRYSISDNNLFHFNKKMFARRRILLKKNRLKRAGHGAKNKLKPISILTEKSERFRKKLIERWACEIADFFIRNKVGTVQMENLEGMKRKEDSYFNIRLRGFWPYAEMQNKIEFKLKQYGIVVRKVAPNNTSKTCSKCGHLNNYFNFEYRKKNKFPHFKCEKCNFKENADYNAALNISNPKLKSTKEGP

SEQ ID NO: 1816 - protein, 726 aa, synthetic construct
SEVEFSHEYWMRHALTLAKRARDEREVPVGAILVLNNRVIGEGWNRAIGLHDPTAHAEIMALRQGGLVMQNHRLIDATLYVTFEPCVMCAGAMIHSRIGRVVFGVRNSKHGAAGSLMNVLDYPGMGHRVEITEGILADECAALLCDFYCMPRQVFNAQKRAQSSINSGGSSGGSSGSETPGTSESVTPESSGGSSGGSAKNTITKTLKLRIVRPYNSAEVEKIVADEKNNREKIALEKNKDKVKEACSKHLKVAAYCTTQVERNACLFCKARRLDDKFYQKLRGQFPDAVFWQEIGEIFRQLQKQAAEIYNQSLIELYYEIFIKGKGIANASSVEHYLSDVCYTRAAELFKNAAIASGLRNKVKSNFRLKELRSMKSGLPTTKSDNFPIPLVKQKGGQYTGFEISSHNDDFIIKIPFGRWQAKKEIDKYRPWEKFDFEQVRKSPKPISLLLSTQRRKRNRGWSKDEGTEAEIRKVMNGDYQTSYIEVKRGSKIGEKSAWMLNLSIDVPKIDKGVDPSIIGGIDVGVKSPLVCAINNAFSRYSISDNDLFRFNKKMFARRRILLGKNRHKRAGHGVKNKLKPITILTEKSGRFRKKLIERWACEIADFFVKNKVGTVQMENLESMKRKEDSYFNIRLRGFWPYAEMQNKIEFKLKQYGIKVRKVAPNNTSKTCSKCGHLNNYFSFEYRKKNKFPHFKCEKCNFKENADYNAALNISNPKLKSTKEEP

SEQ ID NO: 1817 - protein, 726 aa, synthetic construct
SEVEFSHEYWMRHALTLARRARDEREVPVGAVLVLNNRVIGGGWNRTIGLHDPTAHAEIMALRQGGLVMQNCRLADATLYVTFEPCVMCAGAMIHSRIGRVVFGVRNSKRGAAGSLMNVLNYPGMNHRVEIAEGILADECAALLCDFYRMPRRVFNTQKKAQSSINSGGSSGGGSGSDTPSTSESVTPKSSVGSSAGSTKNTITKTLKLRIVRPYNSAEVEKIVADEKDNREKIALEKNKDKVKEACSKHLKVAAYCTTQVERNACLFCKARKLDDKFYQKLRGQFPDAVFWQEVSEIFRQLQKQAAEIYNQSLIELYYEIFIKGKGFANASSVEHYLSDVCYTRAAELFKNAAIASGLRGKVKSNFRLKELKNMKSGLPTTKSDNFPIPLVKQKGGQYTGFEISSHNDDFIIKIPFGRWQAKKEIDRYRPWEKFDFEQVRKNPKPISLLLSTRRRKRNKGWSKDEGTEAEIRRVMNGDYQTSYIEVKRGSKTGEKGAWMLSLSIDVPKIDKGVDPRIIGGIDVGVKSPLVCAINNVLSRYSISDNDLFHFNKKMFARRRILLKKNGHKRAGHGAKNKLKPITIMSEKSRRFRKKLIERWACEIADFFIKNKVGTVQMENLESMKRKEDSYFNIRLRGFWPYAEMQNKIEFKLKQYGIVVRKVAPNNTSKTCSQCGHLNNYFNFEYRKKNKFPYFKCEKCNFKENADYNAALNISNPQLKSTKGEP

SEQ ID NO: 1818 - protein, 726 aa, synthetic construct
SEVEFSHEYWMRHALTLAKRARDGREVPVGAVLVLNNRVIGEGWNRAIGLHDPTAHAEVMALRQGGLVMQNYRLIGATLYVTFEPCAMCAGAMVHSRIGRVVFGVRNSKRGAAGSLMNVLNYPGMDHRVEITGGILADECAALLCDFYRMPRRVFDAQKKAQSSINPGGSSGGSSGSETPGTSESATPESSGGSSGGSAKNIITKTLKLRIVRPYNSAEVEKIVADEKNNREKIALEKNKDKVKEACSKHLKVATYCTTQVERNACLFCKARRLDDKFYQKLRGQFPDAVFWQELGEILRQLQKQAAEIYNQSLIELYYEIFIKGRGFANASSVEHYLSDVCYTRAAELFKNAAIASGLRGKVKSNFRLKELKNMKSGLPTTKSDNFPIPLVKQKGGQYTGFEISNHNGDFIIKIPFGRWQAKKEIDKYRPWEKFDFEQVRKSPKPISLLLSTRRRKRNKGWSKDEGTEAEIRRVMNGDYQTSYIEVKRGSKIGEKSAWMLSLSIDVPKIDKGVDPRIIGGIDVGVKSPLVCAINNVLSRYSISDNDLFHFNKKVFARRRILLKKNRHRRAGHGAKNKLKPITILTEKSKRFRKKLIERWACEIADFFIKNKVGTVQMENLESMKRKEDSYFNIRLRGFWPYAEMQNKIEFKLKQYGIKIRKVAPNNTSRTCSKCGHLNNYFSFEYRKKNKFPHFKCEKCNFKEDADYNAALNISNPELKGTKEEL

SEQ ID NO: 1819 - protein, 726 aa, synthetic construct
SEVEFSHEYWMRHALTLAKRARDGREVPVGAVLVLNNRVIGEGWNRAIGLHDPTAHAEIMALRQGGLVMQNYRLIDATLYVTFEPCVMCAGAMIHSRVGRVVFGVRNSKHGAAGSLMNVLNYPGMNHRVEITEGILADECAALLCDFYRMPRRVFNARRKAQSSIDPGGSSDGGSGSETPGTSESATPESSGGSSGGSAKNTITKTLKLRIVRPYNSAEVEKIVADEKNNREKIALERNKDKVREACNKHLKVASYCTTQVERNACPFCKARKLDDKFYQKLRGQFPDAVFWQELGEILRQLQKQAAEIYNQSLIELYYEIFIKGRGFANASSVEHYLSDVCYTRAAELFKNAAIASGLRGKVKSNFRLKELKNMKSGLPTTKSDNFPIPLVKQKGGQYTGFEISSHNDDFIIKIPFGRWQVKKEIDKYRPWEKFDFEQVRKSPKPISLLLSTQRRKRNKGWSKDEGTEAEIRKVMNGDYQTSYIEVKRGSKIGEKSAWMLSLSIDVPKIDKGVDPSIIGGIDVGVKSPLVCAINNAFCRYSISDNDLFHFNKKMFARRRILLKKSRHKRAGHGAKNKLKPISILTGKSERFRKKLIERWACEIADFFIKNKVGTVQMENLESMKRKEDSYFNIRLRGFWPYAEMQNRIEFKLKQYGIEIRKVAPNNTSKTCSKCGHLNNYFNFEYRKKNKFPHFKCEKCNFKENADYNAALNISNPKLKSTKEEP

SEQ ID NO: 1820 - protein, 726 aa, synthetic construct
SEVEFSHEYWMRHALTLAKRARDEREVPVGAILVLNNRVIGVGWNRAIGLHDPTAHAEIMALRQGGLVTQNYRLINATLYVTFEPCVMCAGAMIHSRIGRVVFGVRNSKHGAAGSLVNVLNYPGMNHRVEITEGILADECAALLCDFYRMPRRVFNAQKKAQSSINSGGSSGGGSGSETPSTSESTTPESSGGSSAGPTKNTITKTLKLRIVRPYNSAEVERTVADEKNNRERIALEKNKDKVKEACSKHLKVAAYCTTQVERNACLFCKARKLDDKFYQKLRGQFPDAVFWQEIGEIFRQLQRQAAEIYNRSLIELYYEIFIKGKGFANASSVEHYLSDVCYTRAAELFKNAAIASGLRSKVRSNFRLKELKNMKSGLPTTKSDNFPIPLVKQKGGQYTGFEISSHNSDFIIKIPFGRWQVKEEIDKYRPWEKFDFEQVRKSPKPISLLLSTQRRKKNKGWSKDEGTEAEIRRVMNGDYQTSYIEVKRGSKIGEKSAWMLNLSIDVPKIDKGVDPSIIGGIDVGVKSPLVCAINNSSSRYSICDNDLFRFNKKMFARRRILLKKNRHKRAGHGAKNKLKPITILTKKSERFRRKLIERWACEVADFFIKNKVGTVQMENLESMKRKEDSYFNIRLRGFWPYAEMQNRIEFKLKQYGIEIRKVAPNNTSKTCSKCGHLNNYFNFEFRKRNKFPHFKCEKCNFKENADYNAALNISNPKLKSTKEEP

SEQ ID NO: 1821 - protein, 726 aa, synthetic construct
SEVEFSHEYWMRHALTLAKRARDEREVPVGAILVLNNRVIGEGWNRAIGLHDPTAHAEIMAMRQGGLVLQNYRLIDATLYVTFEPCVMCAGAMIHSRIGRVVFGVRNNKHGAAGSLVNVLNYPGMNHRVEITEGILADECAALLCDFYRMPRQVFNARKKAQSSINPGGSSGGSSGSETPGTSESATPESSGGSSGSSAKNTITKTLKLRIVRPYNSAEVEKIVADEKNNREKIALEKNKDKVKEACSKHLKVAAYCTTQVERNACLFCKARRLDDKFYQKLRGQFPDAVFWQEIGEIFRQLQKQAAEIYNQSLIELYYEIFIRGKGIANASSVEHYLSDVCYTRAAELFKNAAIASGLRNKVKSNFRLKELRSMKSGLPTTKSDNFPIPLVRQKGGQYTGFEISNHNSDFIIKIPFGRWQAKKEIDKYRPWEKFDFEQVRKSPKPISLLLSTQRRKRNRGWSKDESTEAEIKKVMNGDYQTSYIEVKRGSKVGEKSAWMLNLSIDVPKIDKGVDPSIIGGIDVGVKSPLVCAINNAFSRYSISDNDLFRFNKKMFARRRILLKKSKHKRAGHGARNKLKPITVLTEKSERFRKKLIERWACEIANFFIKNKVGTVQMENLESMKRREDSYFNIRLRGFWPYAEMQNKIEFKLKQYGIEIRKVAPNNTSKTCSKCGHLNSYFNFEYRKKNKFPHFKCEKCNFKENADYNAALNISNPKLKSTKEEP

SEQ ID NO: 1822 - protein, 726 aa, synthetic construct
SEVEFSHEYWMRHALTLAKRARDEREVPVGAVLVLNNRVIGEGWNRAIGLHDPTAHAEIMALRQGGLVMQNYRLVDATLYVTFEPCVLCAGAMVHSRIGRVVFGVRNSKRGAAGSLMNVLNYPGMNHRVEITEGILADECAALLCDFYRMPRQVFNARKKAQSSINPGGSSGGSSGSGTPGTSESATPESSGGSSSGSAKNTITKALKLRIVRPYNSAEVEKIVADEKNNRERIALEKNKDKVKEACSKHLKVAAYCTTQVERNACLFCKARKLDDKFYQKLRGQFPDAVFWQEIGEIFRQLQKQAAEIYNQSLIELYYEIFIKGKGFANASSVEHYLSDVCYTRAAELFKNAAIASGLRGKVKSNFRLKELKNMRSGLPTTKSDNFPIPLVKQKGGQYAGFEISSHNDDFIIKIPFGRWQVKKEIDKYRPWEKFDFEQVRKSPKPISLLLSTRRRKRNKGWSKDEGTEAEIRKVMNGDYQTSYIEVKRGSKIGEKSAWMLNLSIDVPKIDKGVDPSIIGGIDVGVKSPLVCAINNAFGRYSISDNDLFHFNKKMFARRRILLKKNRHKRAGHGTKNKLKPITILTEKSRRFRRKLIERWACEIADFFIKNKVGTVQMESLESMKRKEDSYFNIRLRGFWPYAEMQSKIEFKLKQYGIKIRKVAPNNTSKTCSKCGHLNNYFSFEYRKKNKFPHFKCEKCNFKENADYNAALNISNPKLMSTKVEP

SEQ ID NO: 1823 - protein, 726 aa, synthetic construct
SEVEFSHEYWMRHALTLAKRARDEREVPVGAVLVLNNRVIGEGWNRAIGLHDPTAHAEIMALRQGGLVMQNYRLTDATLYVTFEPCVMCAGAMIHSRIGRVVFGVRNSKHGAAGSLMNVLNYPGMNHRVEITEGILADECAALLCDFYRMPRQVFNARKKAQSSVSSGGSSGGGSGSETPGASESATPESSGGSSGGSAKNTITKTLQLRIVRPYNSAEVEKIVTDEKNNREKIALEKNKGKVKEACSKHLKMASYCTTQVERNACLFCKARRLDDKFYQKLRGQFPDAVFWQELGEILRQLQKQAAEIYNQSLIELYYEIFIKGRGFANASSVEHYLSGVCYTRAAELFKNAAIASGLRGKVKSNFRLKELKNMKSGLPTTKSDNFPIPLVKQKGGQYTGFEISSHNDDFIIKIPFGRWQVKKEIDKYRPWEKFDFEQVRKSPKPISLLLSTQRRKRNKGWSKDEGTEAEIRKVMNGDYQTSYIEVKRGSKIDEKSAWMLNLSIDVPKIDKGVDPSIIGGIDVGVKSPLVCAINNAFSRYSISDNDLFRFNKKMFARRRILLGKNRHKRAGHGVKNKLKPITILTEKSGRFRKKLIERWACEIADFFVKNKVGTVQMENLESMKRKEDSYFNIRLRGFWPYAEMQDKIEFKLKQYGIKVRKVAPNNTSKICSKCGHLNNYFSFEYRKKNKFPHFKCEKCNFKENADYNAALNISNPKLKSTKEEP

SEQ ID NO: 1824 - protein, 726 aa, synthetic construct
SEVEFSHEYWMRHALTLAKRARDEREVPVGAVLVLNNRVIGEGWNRAIGLHDPTAHAEIMALRQGGLVMQNYRLVDATLYVTFEPCVLCAGAMVHSRIGRVVFGVRNSKRGAAGSLMNVLNYPGMNHRVEVTEGILADECAALLCDFYRMPRQVFNARKKVQSSINSGGSSDGGSSSETPGTSESATPESSGGSSGGSAKNTITKTLQLRIVRPYNSTEVEKIVADEKNNREKIALEKNKDKVKEACSKHLKVASYCTTQVERNACLFCKARKLDDKFYQKLRGQFPDAVFWQELGEIFRQLQKQAAEIYNQSLIELYYEIFIKGKGFAIASSVEHYLSCVCYTRAAELFKNAAIASGLRGKVKSNFRLKELKNMKSGLPTTKSDNFPIPLVKQKGGQYTGFEISSHNDDFIIKIPFGRWQAKKEIDKYRPWEKFDFEQVRKSPKPISLLLSTQRRKRNRGWSEDEGTEAEIRKVMNGDYQTSYIEVKRGSKIGEKSAWMLNLSIDVPKIDKGVDPSIIGGIDVGVKSPLVCAINNAFSRYSISDNDLFRFNKKMFARRRILLGKNRHKRAGHGVKNKLKPISILTEKSKRFRKKLIERWACEIADFFVKNKVGTVQMENLESMKRKEDSYFNIRLRGFWPYAEMQNKIEFKLKQYGIKVRKVAPNNTSKTCSKCGHLNNYFSFEYRKKNKFPHFKCEKCNFKENADYNAALNISNPKLKSAKEEP

SEQ ID NO: 1825 - protein, 726 aa, synthetic construct
SEVEFSHEYWMRHALTLAKRARDEREVPVGAILVLNNRVIGEGWNRAIGLHDPTAHAEIMALRQGGLVMRNYRLVDATLYVTFEPCVMCAGAMIHSRIGRVVFGVRNNKHGAAGSLVNVLNYPGMNHRVEITEGILVDECAALLCDFYRMPCQVLNARKKAQSSINPGGSSGGSSGSETPGTSESATPESSGGSSGGSAKNTITKTLKLRIVRPYNSAEVEKIVADEKNNRERIALEKNKDKVKEACSKHLKVASYCTTQVERNACLFCKARKLDDKFYQKLRGQFPDAVFWQELGEIFRQLQKQAAEIYNQSLIELYYEIFIKGKGFANASSVEHYLSDVCYARAAELFKNAAIASGLRGKVKSNFRLKELKNMKSGLPTTKSDNFPIPLVKQKGGQYTGFEISSRNDDFIIKIPFGRWQVKKEIDKYRPWEKFDFEQVRKSPKPISLLLSTQRRKRNKGWSKDEGTEAEIRKVMNGDYQTSYIEVKRGSKIGEKSAWMLNLSIDVPKIDKGVDPSIIGGIDVGVKSPLVCAINNAFSRYSISDNDLFHFNKKMFARRRILLKKNRHKRAGHGAKNKLKPISILTERSKRFRKKLIERWACEIADFFIKNKVGTVQMENLESMKRKEDSYFNIRLRGFWPYAEMQNKIEFKLKQYGIEIRRVAPNNTSRTCSKCGHLNNYFNFEYRKKNKFPHFKCEKCNFKENADYNAALNISNPKLKSIKEEP

SEQ ID NO: 1826 - protein, 726 aa, synthetic construct
SEVEFSHEYWMRRALTLAKRARDEREVPVGAVLVLNNRVIGVGWNRAVGLHDPTAHAEIMALRQGGLVMQNYRLVEATLYVTFEPCIMCAGAMIHSRIGRVVFGVRNSKRGAAGSLMNVLNYPGMNHRVEITEGILADECAALLCDYYRMPRQVFNARKKAQSSINPGGSSGGSGGSETPGTSESTTPEGSGSSSGSSAKNTITKTLKLRIVRPYNSAEVEKIVADEKNNREKIALEKNKDKVKEACSKHLKVAAYCTTQVERNACLFCKARKLDDRFYQKLRGQFPDAVFWQEVGEIFRQLQKQAAETYNQSLIELYYEIFIKGKGFANASSVEHYLSDVCYTRAAELFKNAAIASGLRGKVKSNFRLKELKNMKSGLPTTKSDNFPIPLVKQKGGQYTGFEISNHNSDFIIKIPFGRWQVKKEINKYRPWEKFDFEQVRKGPKPISLLLSTQRRKRNKGWSKDEGTEAEIRKVMNGDYQTSYIEVKRGSKIGEKSAWMLSLSIDVPKIDKGVDPSIIGGIDVGVKSPLVCAINNAFSRYSISDNDLFRFNKKMFARRRILLKKNRHKRAGHGAKNKLKPITILTEKSGRFRKKLIERWACEIADFFIKNKVGTVQMENLESMKRKEDSYFNIRLRGFWPYAEMQNKIELKLKQYGIKIRKVAPNNTSKTCSKCGHLNDYFNFEYRKKNKFPHFKCEKCNFKEDADYNAALNISNPKLKGTKEEP

SEQ ID NO: 1827 - protein, 725 aa, synthetic construct
SEVEFSHEYWMRHALTLAKRARDEREVPVGAVLVLNNRVIGEGWNRAIGLHDPTAHAEIMALRQGGLVMQNYRLIDATLYVTFEPCVMCAGAMIHSRIGRVVFGVRNSKHGAAGSLVNVLNYPGMNHRVEITEGILADECAALLCDFYRMPRQVFNARKKAQSSINPSGLSGGSSGSVTPGTSESATPESSGGGFGGSAKNTITKTLQLRIVRPYNSAEVEKIVADEKDNREKTALEKNKDKVKEACSKHLKVASYCTTQVERNTCLFCKARKLDDKFYQKLRGQFPDAVFWQELGEIFRQLQKQAAEIYNQSLIELYYEIFIKGKGLANASSVEHYLSDVCYTRAAGLFKNAAIASGLRGKVKSNFKLKELKSMKSGLPSTKSDNFPIPLVKQRGGQYTGFEISSHNDDFIIKIPFGRWQAKKEIDKYRPWEKFDFEQVRKSPKPISLLLSTQRRKRNRGWSKDEGTEAEIRKVMNGDYQTSYIEVKRGSKIGEKSAWMLNLSIDVPKIDKGVDPSIIGGIDVGVKSPLVCAINNAFSRYSISDNDLFRFNKKMFARRRILLGKNRHKRAGHGTKNKLKPITILTEKSGRFRKKLIERWACEIADFFVKNKVGTVQMENLESMKRKEDSYFNIRLRGFWPYAEMQNKIEFKLKQYGIVVRKVAPNNTSKTCSKCGHLNNYFNFEYRKKNKFPHFKCEKCNFKENADYNAALNISNPKLKSTEEP

SEQ ID NO: 1828 - protein, 726 aa, synthetic construct
SEVEFSHEYWMRHALTLAKRARDEREVPVGAVLVLNNRVIGEGWNRAIGLHDPTAHAEIMALRQGGLVLQNYRLVDATLYVTFEPCVLCAGAMVHSRIGRVVFGARNSKRGAAGSLMNILNYPGMNHRVEITGGVLADECAALLCDFYRMPRQVFNAQKKAQSSINPGGSSGGSSGGKAPGTSESATLESSGGSSSGSAKNSITKTLKLRIVRPYNSAEVEKIVADEKNNREKIALEKNKGKVEEACSKHLKVAAYCTTQVERNACLFCKARKLDDRFYQKLRGQFPDAVFWQEIGEIFRQLQKQAAEIYNQSLIELYYEIFIEGKGSANARSVEHYLSDVCYTRAAELFKNAAIASGLRNKIKSNFRLKELRNMKSGLPTTKSDNFPIPLVRQKGGQYTGFEISNHDGDFIIKIPFGRWQVKKEINKHRPWEKFDFEQVRKSPKPISLLLSTQRRKRNKGWSKDEGTEAEIKKVMNGGYQISYIEVKRGSKIGEKNAWTLNLSVDVPKIDKGVDPSIIGGIDVGVKSPLVCAINNALSRYSISDNDLFHFNKKVFARRRILLKKNRHRRAGHGAKNKLKPITILTEKSKRFRKKLIERWACEIADFFIKNKVGIVQMENLESMKRREDSYFNIRLRGFWPYAEMQNKIEFKLKQYGIEIRKVAPNNTSKTCSRCGHLNNYFNFEYRRKNKFPHFKCEKCSFKENADYNAALNISNPKLKSTKEKP

SEQ ID NO: 1829 - protein, 726 aa, synthetic construct
SEVEFSHEYWMRHALTLAKRARDEREVPVGAVLVLNNRVIGEGWNRAIGLHDPTAHAEIMALRQGGLVTQNYRLIDATLYVTFEPCVMCAGAMVHSRIGRVVFGVRNSKRGAAGSLMNVLDYPGMGHRVEITEGILADESAALLCDFYRMPRQVFNARKRAQSSINPGGSSGGSGGSETPGTSESATPESSGGSSGSSAKNTITKTLKLRIVRPYNSAEVEKIVADEKNNREKIALEKNKDKVKEACSKHLKVAAYCTTQVERNACLFCKARRLDDKFYQKLRGQFPDAVFWQEIGEIFRQLQKQAAEVYNQSLVELYYEILIKGKGIANASSVEHYLSDVCYTRAAELFKNAAIASGLRNKIKSNFRLKELRNMKSGLPTTKSDNFPIPLVRQKGGQYTGFEISNHDGDFIIKIPFGRWQVKKEINKHRPWEKFDFEQVRKSPKPISLLLSTQRRKRNKGWSKDEGTEAEIRKVMNGDYQTSYIEVKRGSKIGEKSAWMLNLSIDVPKIDKGVDPSIIGGIDVGVKSPLVCAINNAFSRYSISDNDLFHFNKKMFARRRILLKKNRHRRAGHGAKNKLKPITILTEKSRRFRKKLIERWACEIADFFIKNKVGTVQMENLESMKRREDSYFNIRLRGFWPYAEMQNKIEFKLKQYGIEVRKVAPNNTSKTCSKCGHLNSYFNFEYRKKNKFPHFKCEKCNFKEDADYNAALNISNPKLKSTKEEP

SEQ ID NO: 1830 - protein, 726 aa, synthetic construct
SEVEFSHEYWMRHALTLAKRARDEREVPVGAVLVLNNRVIGEGWNRAIGLHDPTAHAEIMALRQGGLVMQNYRLTDATLYVTFEPCVMCAGAMIHSRIGRVVFGVRNSKRGAAGSLMNVLNYPGMNHCVEITEGILVDECAALLCDFYRMPRQVLNAQKKAQSSISSGGSSGGSSCSETPGASESVTPESSGGSSGGSAKNTITKTLKLRIVRPYNSAEVEKIVADEKNNREKIALEKNKDKVKEACSEHLKVAAYCTTQVERNACLFCKARKLDDKFYQKLRGQFPDAVFWQELGEIFRQLQKQAAEIYNQSLIELYYVIFIKGKGLANASSVEHYLSDVCYTRAAELFKNAAIASGLRGKVKSNFKLKELKSMKSGLPSTKSDNFPIPLVKQRGGQYTGFEISSHNDDFIIKIPFGRWQAKKEIDKYRPWEKFDFEQVRKSPKPISLLLSTQRRKRNRGWSKDEGTEAEIRKVMNGDYQTSYIEVKRGSKIGEKSAWMLNLSIDVPKIDKGVDPSIIGGIDVGVKSPLVCAINNAFSRYSISDNDLFRFNKKMFARRRILLGKNRHKRAGHGVKNKLKPITILTEKSGRFRKKLIERWACEIADFFVKNKVGTVQMENLESMKRKEDSYFNIRLRGFWPYAEMQNKIEFKLKQYGIKVRKVAPNNTSKTCSKCGHLNNYFSFEYRKKNKFPHFKCEKCNFKENADYNAALNISNPKLKSTKEEP

SEQ ID NO: 1831 - protein, 725 aa, synthetic construct
SEVEFSHEYWMRHALTLAKRARDEREVPVGAVLVLNNRVIGEGWNRAIGLHDPTAHAEIMALRQGGLVMQNYRLTDATLYVTFEPCVMCAGAMIHSRIGRVVFGVRNNKHGAAGSLVNVLNYPGMNHRVEITEGILADECAALLCDFYRMPRQVFNARKKARSNINSGCSSGGSSGSETPGTSESATPESSGSSSGGSTKNTITKTLKLRIVRPYNSAEVEKIVADEKNNREIALEKNKDKVKEACSKHLKVAAYCTTQVERNACLFCRARRLDDKFYQKLRGQFPDAVFWQEIGEIFRQLQRQAAEIYNQSLVELYYEIFIKGKGIANASSVEHYLSDVCYTRAAELFKNAAIASGLRNKIKSNFRLKELRNMKSGLPTTKSDNFPIPLVRQKGGQYTGFEISNHNSDFIIKIPFGRWQVKKEIDKYRPWEKFDFAQVRKSPKPISLLLSTQRRKRNKGWSKDEGTEAEIRKVMNGDYQTSYIEVKRGGKIGEKSAWMLSLSIDVPKIDKGVDPCITGGIDVGVKSPLVCAINNAFSRYSISDNDLFRFNKKMFARRRILLKKNRHKRAGHGAKNKLKPISILTGKSERFRKKLIERWACEIADFFIKNKVGTVQMENLESMKRKEDSYFNIRLRGFWPYAEMQNKIEFKLKQYGIEIRKVAPNNTSKTCSKCGHLNNYFNFEYRKKNKFPHFKCEKCNFKENADYNAALNISNPKLKSTKEEP

SEQ ID NO: 1832 - protein, 726 aa, synthetic construct
SEVEFSHEYWMRHALTLAKRARDEREVPVGAILVLNNRVIGEGWNRAIGLHDPTAHAEIMALRQGGLVMQNYRLIDATLYVTFEPCVMCAGAMIHSRIGRVVFGVRNSKHGAAGSLVNVLNYPGMNHRVEITEGILADECAALLCDFYRMPRQVFNARKKAQPSINSGGSSGGSSGSVTPGTSESATPESSGGSSGGSAKNTITKTLKLRIVRPYNSAEVEKIVADEKNSREKIALERNKDKVKEACSEHLKVAAYCTTQVERNACLFCKARKLDDRFYQKLRGQFPDAVFWQETGEIFRQLQRQAAEIYNQSLIELYYEIFIRGKGFANASSVEHYLSDVCYTRAAELFKNAAIASGLRGKVKSNFRLKELKNMKSGLPTTKSDNFPIPLVKQKGGQYTGFEISSHNDDFIIKIPFGRWQVRKEIDKYRPWEKFDFEQVRKSPKPISLLLSTQRRKRNKGWSKDEGTEAEIRKVMNGDYQTSYIEVKRGSKIGEKSAWMLSLSIDVPKIDKGVDPSIIGGIDVGVKSPLVCAINNAFSRYSISDNDLFRFNKKVFARRRILLKKNRHKRAGHGTKNKLKPITILTEKSGRFRKKLIERWACEIANFFIKNKVGTVQMEDLESMKRKEDSYFNIRLRGFWPYAEMQNKIEFKLKQYGIKIRKVAPNNTSKTCSKCGHLNNYFSFEYRKKNKFPHFKCEKCSFKEDADYNAALNISNPKLKSTKEEP

SEQ ID NO: 1833 - protein, 726 aa, synthetic construct
SEVEFSHEYWMRHALTLARRARDEREVPVGAILVLNNRVIGEGWNRAIGLHDPTAHAEIMALRQGGLVMQNYRLIDATLYVTFEPCVMCAGAMIHSRIGRVVFGVRNSKRGAAGSLMNVLNYPGMNHCVEITEGILVDECAALLCDFYRMPRQVLNAQKKAQSSISPGGSSGGSSGSETPGTSESTTPGSSGGSSGGSAKDTITKTLKLRIVRPYNSAEVEKIVADEKNNREKIALEKNKDKVKEACSKHLKVASYCTAQVERNACLFCKARKLDDKFYQKLRGQFPDAVFWQELGEIFRQLQKQAAEIYNQSLIELYYEIFIKGKGFANASSVEHYLSDVCYTRAAELFKNAAIASGLRGKVKSNFRLKELKNMKSGLPTTKSDNFPIPLVKQKGGQYTGFEISSHNDDFIIKIPFGRWQVKEEIDKYRPWEKFDFEQVRKNPKPISLLLSTQRRKRNKGWSKDEGTEAEIRKVMNGDYQTSYIEVKRGSKIGEKSAWMLNLSIDVPKIDKGVDPSIIGGIDVGVKSPLVCAINNAFSRYSISDNDLFRFNKKVFARRRILLKKNRHKRAGHGTKNKLKPITILTERSGRFRKKLIERWACEIANFFIKNKVGTVQMENLESMKRKEDSYFNIRLRGFWPYAEMQNKIEFKLKQYGIKIRKVAPNNTSKTCSKCGHLNNYFSFEYRKKNKFPRFKCEKCNFKEDADYNAALNISNPKLKSTKEEP

SEQ ID NO: 1834 - protein, 726 aa, synthetic construct
SEVEFSHEYWMRHALTLAKRARDEREVPVGAILVLNNRVIGEGWNRAIGLHDPTAHAEIMALRQGGLVMQNYRLTDATLYATFEPCVMCAGAMIHSRIGRVVFGVRNSKHGAAGSLMNVLNYPGMNHRVEITEGILADECAGLLCDFYRMPRQVFSARKKAQSSINPGGSSGGSSGGKAPGTCESATLESSGGSSGDSAKNSITKTLKLRIVRPYNSAEVEKIVADEKNNREKIALEKNKGKVEEACSRHLKVATYCTTQVERNACLFCKARKLDDKFYQKLRGQFPDAVFWQEIGEIFRQLQKQAAEIYNQSLIELYYEIFIKGKGFANASSAEHYLSDVCYTRAAELFKNAAIASGLRGKVKSNFRLKELKNMKSGLPTTKSDNFPIPLVKQKGGKYTGFEISSHNDDFIIKIPFGRWQVKKEIDKYRPWEKFDFEQVRKSPKPISLLLSTQRRKRNKGWSKDEGTEAEIRKVMNGDYQTSYIEVKRGSKIGEKSAWMLNLSIDVPKIDKGVDPSIIGGIDVGVKSPLVCAINNAFSRYSISDNDLFHFNKKMFARRRILLKKNRHKRAGHGAKNKLKPISILTEKSKRFRKKLIERWACEIADFFIKNKVGTVQMENLESMKRKEDSYFNIRLRGFWPYAEMQNKIEFKLKQYGIEIRKVAPNNTSKTCSKCGHLNNYFNFEYRKKNKFPHFKCEKCNFKENADYNAALNISNPKLKSTKEEP

SEQ ID NO: 1835 - protein, 726 aa, synthetic construct
SEVEFSHEYWMRHALTLAKRARDDREVPVGAVLVLNNRVIGEGWNRAIGLHDPTAHAEIMALRQGGLVMQNYRLIDATLYVTFEPCVMCAGAMIHSRIGRVVFGVRNSKHGAAGSLMNVLNYPGMNHRVEITEGILADECAALLCDFYRMPRQVFNARKKAQSSINPGGSSGGSSGSETPGTSESATPESSGGSSGGSAKNTITKTLKLRIVRPYNSAEVEKIVADEKNNRERIALEKNKDKVKEACSKHLKVAAYCTTQVERNACLFCKARKLDDKFYQKLRGQFPDAVFWQEVGGIFRQLQKQAAEIYNQSLIELYYEIFIKGKGFANASSVEHYLSDVCYARAAELFKNAAIASGLRGKVKSNFRLKELKNMKSGLPTTKSDNFPIPLVKQKGGQYTGFEISNHNDDFIIKIPFGRWQVKEEIDKYRPWEKFDFEQVRKNPKPISLLLSTQRRKGNKGWSKDEGTEAEIRKVMNGDYQTSYIEVKRGSKIGEKSAWMLNLSIDVPKIDKGVDPSIIGGIDVGVKSPLVCAINNAFSRYSISDNDLFRFNKKVFARRRILLGKNRHKRAGHGVKNKLKPITTLTEKSGRFRKKLIERWACEIADFFVKNKVGTVQMENLESMKRREDSYFNIRLRGFWPYAEMQNKIEFKLKQYGIKVRKVAPNNTSKTCSKCGHLNNYFSFEYRKKNKFPHFKCEKCNFKEDADYNAALNISNPKLKSTKEEP

SEQ ID NO: 1836 - protein, 726 aa, synthetic construct
SEDEFSHEYWMRHALTLAKRARDGREVPVGAVLVLNNRVIGEGWNRAIGLHDPTAHAEIMALRQGGLVMQNYRLIDATLYVTFEPCVMCAGAMVHSRIGRVVFGVRNGKRGAAGSLMNVLDYPGMGHRVEITEGILADECAALLCDFYCMPRQVFNAQKRAQSSINSGGSSGGSSGSETPGTSESATPGSSGGSSSGSAKNTITKTLKLRIVRPYNSTEVERIVADEKNNREKIALEKNKDKVKEACSKHLKVASYCTTQVERNACLFCKARKLDDRFYQKLRGQFPDAVFWQETGEIFRQLQRQAAEIYNQSLIELYYEIFIKGKGFANASSVEHYLSDVCYTRAAELFKNAAIASGLRGKVKSNFRLKELKNMKSGLPTTKSDNFPIPLVKQKGGQYTGFEISSHNDDFIIKIPFGRWQVKKEIDKYRPWEKFDFEQVRKSPKPISLLLSTQRRKRNKGWSKDEGTEAEIRKVMNGDYQTSYIEVKRGSKTGEKSAWMLNLSIDVPKIDKGVDPSIIGGIDVGVKSPLVCAINNALSRYSISDNDLFRFNKKMFARRRILLKKNRHKRAGHGAKNKLKPISILTGKSERFRKKLIERWACEIADFFIKNKVGTVQMENLESMKRKEDSYFNIRLRGFWPYAEMQNKIEFKLKQYGIEIRKVAPNNTSKTCSKCGHLNNYFNFEYRKKNKFPHFKCEKCNFKENADYNAALNISNPRLKSTKEEP

SEQ ID NO: 1837 - protein, 726 aa, synthetic construct
SGVEFSHEYWMRHALTLAKRARDEREVPVGAILVLNNRVIGEGWNRAIGLHDPTAHAEIMALRQGGLVMQNYRLIDATLYVTFEPCAMCAGAMVHSRIGRVVFGVRNSKRGAAGSLMNVLNYPGMDHRVEITGGILADECAALLCDFYRMPRRVFNAQKKAQPSINSGGSSGGSSGSVTPGTSESATPESSGGGFGGSAKNTITKTLQLRIVRPYNSAEVEKIVADEKNNREKIALEKNKDKVKEACSKHLKVASYCTTQVERNACLFCKARKLDDKFYQKLRGQFPDAVFWQELGEIFRQLQKQAAEIYNQSLIELYYEIFIKGKGLANASSVEHYLSDVCYTRAAELFKNAAIASGLRGKVKSNFRLKELKNMKSGLPTTKSDNFPIPLVKQKGGQYTGFEISSHNDDFIIKIPFGRWQVKKEIDKYRPWEKFDFEQVRKSPKPISLLLSTRRRKRNKGWSKDEGTEAEIRKVMNGDYQTSYIEVKRGSKIGEKSAWMLNLSIDVPKIDKGVDPSIIGGIDVGVKSPLVCAINNAFGRYSISDNDLFHFNKKMFARRRILLKKNRHKRAGHGTKNKLKPITILTEKSGRFRKKLIERWACEIANFFIKNKVGTVQMENLESMKRKEDSYFNIRLRGFWPYAEMQNKIEFKLKQYGIEIRKVAPNNTSKTCSKCGHLNNYFNFEYRKMNKFPHFKCEKCNFKENADYNAALNISNPKLKSTKEEP

SEQ ID NO: 1838 - protein, 726 aa, synthetic construct
SEVEFSHEYWMRHALTLAERARDAREVPVGAILVLNNRVIGEGWNRAIGQHDPTAHAEIMALRQGGLVMQNYRLIDATLYVTFEPCVMCAGAMIHSRIGRVVFGVRNSKHGAAGSLMNVLNYPGMNHRVVITEGILADECAALLCDFYRMPRQVFNGRKKAQSSINSGGSSGGSSGSETPGTSESATPESSGGSSSGSTKNTITKTLKLRIVRPYNSTEVEKIVADEKNNREKIALEKNKDKVKEACSRHLKVAAYCTTQVERNACLFCKARKLDDKFYQKLRGQFPDAVFWQEIGEIFRQLQKQAAEIYNQSLIELYYEIFIKGKGFANASSVEHYLSDVCYARAAELFKNAAIASGLRGKVKSNFRLKELKNMKSGLPTTKSDNFPIPLVKQKGGQYTGFEISNHNDDFIIKIPFGRWQVKEEIDKYRPWEKFDFEQVRKNPKPISLLLSTQRRKGNKGWSKDEGTEAEIRKVMNGDYQTSYIEVKRGSKIGEKSAWMLNLSIDVPKIDKGVDPSIIGGIDVGVKSPLVCAINNAFSRYSISDNDLFHFNKKVFARRRILLKKNRHRRAGHGAKNKLKPITILTEKSKRFRKKLIERWACEIADFFIKNKVGTVQMENLESMKRKEDSYFNIRLRGFWPYAEMQNKIEFKLKQYGIKIRKVAPNNTSRTCSKCGHLNNYFSFEYRKKNKFPHFKCEKCNFKEDADYNAALNISNPKLKGTKEEP

SEQ ID NO: 1839 - protein, 726 aa, synthetic construct
SEVEFSHEYWMRHALTLAKRARDEREVPVGAVLVLNNRVIGEGWNRAIGLHDPTAHAEIMALHQGGLVMQNYRLIDATLYVTFEPCVMCAGAMIHSRIGRVVFGARNSKRGAAGSLMNVLSYPGMNHRVEITEGILADECAALLCDFYRMPRRVFNAQKKAQSSINSGGSSGGGSSSDTPSTSESTTPESSGGSSGGSAKNTITKTLKLRIVRPYNSAEVEKIVADEKNNREKIALEKNKDKVKEACSKHLKVAAYCTTQVERDACLFCKARRLDDKFYQKLRGQFPDAVFWQELGEILRQLQKQAAEIYNQSLIELYYEIFIKGRGFANASSVEHYLSDVCYTRAAELFKNAAIASGLRGKVKSNFRLKELKNMKSGLPTTKSDNFPIPLVKQKGGQYTGFEISSHNDDFIIKIPFGRWQVKKEIDKYRPWEKFDFEQVRKSPKPISLLLSTQRRKRNKGWGKDEGTEAEIRKVMNGDYQTSYIEVKRGSKSGEKSAWMLNLSIDVPKIDKGVDPSIIGGIDVGVKSPLVCAINNAFSRYSISDNDLFRFNKKMFARRRILLKKNRHKRAGHGAKNKLKPISILTGKSERFRKKLIERWACEIADFFIKNKVGTVQMENLESMKRKEDSYFNIRLRGFWPYAEMQNKIEFKLKQYGIEIRKVAPNNTSKTCSKCGHLNNYFNFEYRKKNKFPHFKCEKCNFKENADYNAALNISNPKLKSTKEEP

SEQ ID NO: 1840 - protein, 726 aa, synthetic construct
SEVEFSHEYWMRHALTLAERARDEREVPVGAVLVLNNRVIGEGWNRAIGLHDPTAHAEIMALRQGGLVMQNYRLIGATLYVTFEPCVMCAGAMIHSRIGRVVYGVRNGKRGAAGSLMNVLNYPGMNHRVEITEGILADECAALLCDFYRMPRQVLNAQKRAPSSINPGGPSGGSSSGETPGTSKSATPESSGGGSGGSAKSTITKTLQLRIVRPYNSAEVEKIVADEKNNREKIALEKNKDKVREACSKHLKVASYCTTQVERNACPFCKARKLDDKFYQKLRGQFPDAVFWQEIGEIFRQLQKQAAEIYNQSLIELYYEIFIKGKGFANASSAEHYLSDVCYTRAAELFKNAAIASGLRNKVKSNFRLKELRSMKSGLPTTKSDNFPIPLVRQKGGQYTGFEISSHNDDFIIKIPFGRWQVKKEIDKYRPWEKFDFEQVRKSPKPISLLLSTQRRKRNKGWSRDEGTEAEIRKVMNGDYQTSYIEVKRGSKTGEKSAWMLNLSIDVPKIDKSVDPSIIGGIDVGVKSPLVCAINNAFSRYSISDNDLFRFNKKMFARRRILLKKNRHKRAGHGAKNKLKPITILTEKSKRFRKKLIERWACEIADFFIKNKVGTVQMENLESMKRKEDSYFNIRLRGFWPYAEMQNKIEFKLKQYGIKIRKVAPNNTSRTCSKCGHLNNYFSFEYRKKNKFPHFKCEKCNFKEDADYNAALNISNPKLKGTKEEL

SEQ ID NO: 1841 - protein, 726 aa, synthetic construct
SEVEFSHEYWMRHALTLAKRARDEREVPVGAVLVLNNRVIGVGWNRAVGLHDPTAHAEIMALRQGGLVMQNYRLVDATLYVTFEPCVLCAGAMVHSRIGRVVFGVRNSKRGAAGSLMNVLNYPGMNHRVEITEGILADECAALLCDFYRMPRQVFNARKKARSNINSGGSSGGSSGSEALGTSESATPESSGGSSGGSAKNTITKTLKLRIVRPYNSAEVEKIVADEKNNREKIALEKNKDKVKEACGEHLKVAAYCTTQVERNACLFCKARKLDDKFYQKLGGQFPDAVFWQEIGEIFRQLQRQAAEIYNQSLIELYYEIFIKGKGFANASSVEHYLSDVCYTRAAELFKNAAIASGLRGKVKSNFRLKELKNMRSGLPTTKSDNFPIPLVRQKGGRYTGFEISNHNGDFIIKIPFGRWQVKKEINKHRPWEKFDFEQVRKSPKPISLLLSTQRRKRNKGWSKDEGTEAEIRKVMNGDYQTSYIEVKRGSKIGEKSAWMLSLSIDVPKIDKGVDPSIIGGIDVGVKSPLVCAINNAFNRYSISDNNLFHFNKKMFARRRILLKKNRHKRAGHGAKNKLKPISILTEKSKRFRKKLIERWACEIADFFIKNKVGTVQMENLEGMKRKEDSYFNIRLRGFWPYAEMQNKIEFKLKQYGIVVRKVAPNNTSKTCSKCGHLNNYFNFEYRKKNKFPHFKCERCNFKEDADYNAALNISNPKLKSTKEEP

SEQ ID NO: 1842 - protein, 726 aa, synthetic construct
SEVEFSHEYWMRHALTLAKRARDEREVPVGAVLVLNNRVIGEGWNRAIGLHDPTAHAEIMALRQGGLVMQNYRLIDATLYVTFEPCVMCAGAMIHSRIGRVVFGVRNSKHGAAGSLVNVLNYPGMNHRVEITEGILADECAALLCDFYRMPRQVFNAQKKARSCINPGGSSGGSSGSETPGTSESATPESSGGSSGGSAKNTITKTLKLRIVRPYNSAEVEKIVADEKDNRERIALEKNKGKVKEACSKHLKVAAYCTTQVERNACLFCKARKLDDKFYQELRGRFPDAVFWQEIGEIFRQLQKQAAEIYNQSLIELYYEIFIKGKGIANASSVEHYLSDVCYTRAAELFKNAAIASGLRSKVRSNFRLKELKNMKSGLPTTKSDNFPIPLVKQKGGQYTGFEISNHNGDFIIKIPFGRWQAKKEIDKYRPWEKFDFEQVRKSPKPISLLLSTQGRKRNRGWGKDEGTEAEIKKVMNGDYQTSYIEVKRGSKVGEKSAWMLNLSIDVPKIDKGVDPSIIGGIDVGVKSPLVCAINNAFSRYSISDNDLFRFNKKMFARRRILLKKNRHKRAGHGAKNKLKPISILTERSERFRKKLIERWACEIADFFIKNKVGTVQMENLESMKRKGDSYFNIRLRGFWPYAEMQNKIEFKLKQYGIKIRKVAPNNTSKTCSKCGHLNNYFSFEYRKKNKFPHFKCEKCNFKEDADYNAALNISNPKLRSTKEEP

SEQ ID NO: 1843 - protein, 726 aa, synthetic construct
SEDEFSHEYWMRHALTLAKRARDGREVPVGAVLVLNNRVIGEGWNRAIGLHDPTAHAEIMALRQGGLVMQNYRLIDATLYVTFEPCVMCAGAMVHSRIGRVVFGVRNSKRGAAGSLMNVLNYPGMNHRVEITEGILVDECAALLCDFYRMPRQVFNAQKRAQSSINSGGSSGGSSGSETPGTSESATPESSGASSGGSAKNTITKTLQLRIVRPYNSAEVEKIVADEKNNREKIALEKNKGKVKEACSKHLKVASYCTTQVERNACPFCKARKLDDKFYQKLRGQFPGAVFWQELGEIFRQLQKQAAEIYNQSLIELYYKIFIKGKGLANASNVEHYLSDVCYTRAAELFKNAAIASGLRGKVKSNFKLKELKSMKSGLPSTKSDNFPIPLVKQKGGQYTGFEISSHNDDFIIKIPFGRWQVKKEIDKYRPWEKFDFEQVRKSPKPISLLLSTQRRKRNKGWSKDEGTEAEIRRVMNGDYQTSYIEVKRGSKIGEKSAWMLNLSIDVPKIDKGVDPSIIGGIDVGVKSPLVCAINNAFSRYSISDNDLFRFNKKMFARRRILLGKNRHKRAGHGVKNKLKPITILTEKSGRFRKKLIERWACEIADFFVKNKVGTVQMENLESMKRKEDSYFNIRLRGFWPYAEMQNKIEFKLKQYGIEIRKVAPNNTSRTCSKCGHLNNYFNFEYRKKNKFPHFKCEKCNFKENADYNAALNISNPKLKSTKEEP

SEQ ID NO: 1844 - protein, 726 aa, synthetic construct
SEVEFSHEYWMRHALTLAKRARDEREVPVGAVLVLNNRVIGEGWNRAIGLHDPTAHAEIMALRQGGLVLQNYRLADATLYVTFEPCVMCAGAMIHSRIGRVVFGVRNGKRGAAGSLMNVLNYPGMNHCVEITEGILMDECAALLCDFYRMPRQVLIAQKKVQSSISSGGSSGGSSGSETPGACESVTPKSSGGSSAGSTKNTITKTLKLRIVRPYNSAEVEKIVSDEKNNREKIALERNKDKVKEACSKHLKVAAYCTTQVERNACLFCKARKLDDKFYQKLRGQFPDAVFWQEIGEIFRQLQKQAAEIYNQSLIELYYEIFIKGRGFANASSVEHYLSDVCYTRAAELFKNAAIASGLRGKVKSNFRLKELKSMKSGLPSTKSDNFPIPLVKQKGGQYTGFEISSHNDDFIIKIPFGRWQVKEEIDKYRPWEKFDFEQVRKNPKPICLLLSTQRRKGNKGWSKDEGTEAEIRKVMNGDYQTSYIEVKRGSKIGEKSAWMLSLSIDVPKIDKGVDPSIIGGIDVGVKSPLVCAINNAFCRYSISDNDLFHFNKKMFARRRILLKKSRHKRAGHGAKNKLKPISILTEKSKRFRKKLIERWACEIADFFIKNKVGTVQMENLEGMKRKEDSYFNIRLRGFWPYAEMQNKIEFKLKQYGIEIRKVAPNNTSRTCSKCGHLNNYFNFEYRKKNKFPHFRCEKCNFKEDADYNAALNISNPKLKSTKEEP

SEQ ID NO: 1845 - protein, 726 aa, synthetic construct
SEVEFSHEYWMRHALTLAKRARDEREVPVGAVLVLNNRVIGEGWNRAIGLHDPTAHAEIMALRQGGLVMQNYRLIDATLYVTFEPCVMCAGAMIHSRIGRVVFGVRNSKHGAAGSLVNVLNYPGMNHRVEITEGILADECAALLCDFYRMPRRVFNARMKAQSSISPGGSSGGSSGSETPSTSESATPESSGGSSGGSAKNTITKTLQLRIVRPYNSAEVEKIVADEKNNREKIALEKNKDKVKEACSKHLKVAAYCTTQVERNACLFCKARRLDDKFYQKLRGQFPDAVFWQEVGEIFRQLQKQAAEIYNQSLVELYYEIFIKGKGIANASSVEHYLSDVCYTRAAELFKNAAIASGLRGKVKSNFRLKELKNMKSGLPTTKSDNFPIPLVKQKGGQYTGFEISSHNGDFIIKIPFGRWQVKKEIDKYRPWEKFDFEQVRKSPKPISLLLSTQRRKRNKGWSKDEGTEAEIRKVMNGDYQTSYIEVKRGSKIGEKSAWMLNLSIDVPKIDKGVDPSIIGGIDVGVRSPLVCAINNAFSRYSISDNDLFHFNKKMFARRRILLKKNRHKRAGHGVRNKLKPITALTEKSERFRKKLIERWACEIANFFIKNKVGTVQMENLESMRRKEDSYFNIRLRGFWPYAEMQNKIEFKLKQYGIEIRKVAPNNTSKTCSKCGHLNNYFSFEYRKKNKFPHFRCEKCNFKENADYNAALNISNPKLKSTKEEP

SEQ ID NO: 1846 - protein, 726 aa, synthetic construct; identical to SEQ ID NO: 684

SEQ ID NO: 1847 - protein, 726 aa, synthetic construct
SEVEFSHEYWMRHALTLAKRARDEREVPVGAILVLNNRVIGEGWNRAIGLHDPTAHAEIMALRQGGLVMQNYRLIDATLYVTFEPCVMCAGAMIHSRIGRVVFGVRNNKHGAAGSLVNVLNYPGMNHRVEITEGILADECAALLCDFYRMPRQVFNARKKAQSSINPGGSSGGSSGSETPGTSESATPESSGGSSGSSAKNTITKTLKLRIVRPYNSAEVEKIVADEKNNREKIALEKNKDKVKEACSKHLKVAAYCTTQVERNACLFCKARKLDDKFYQKLRGQFPDAVFWQEIGEIFRQLQKQAAEIYNQSLIELYYEIFIKGRGFANASSVEHYLSDVCYTRAAELFKNAAIASGLRGKVKSNFRLKELKNMKSGLPTTKSDNFPIPLVKQKGGQYTGFEISSHNDDFIIKIPFGRWRVKKEIDKYRPWEKFDFEQVRKSPKPISLLLSTQRRKRNKGWSKDEGTEAEIRKVMNGDYQTSYIEVKRGSKIGEKSAWMLNLSIDVPKIDKGVDPSIIGGIDVGVKSPLVCAINNAFSRYSISDNDLFHYNKKMFARRRILLKKNRHKRAGHGAKNKLKPITILTEKSVRFRKKLIERWACEIADFFIKNKVGTVQMENLESMKGKEDSYFNIRLRGFWPYAEMQNKIEFKLKQYGIEIRKVAPNNTSKTCSKCGHLNNYFNFEYRKKNKFPHFKCEKCYFKEDADYNAALNISNPRLKSTKEEP

SEQ ID NO: 1848 - protein, 726 aa, synthetic construct
SEDEFSHEYWMRHALTLAKRARDGREVPVGAVLVLNNRVIGEGWNRAIGLHDPTAHAEIMALRQGGLVMQNYRLIDATLYVTFEPCVMCAGAMVHSRIGRVVFGVRNSKRGAAGSLMNVLDYPGMGHRVEITEGILADECAALLCDFYCMPRQVFNARKKAQSSINTGGSSGGSGGSEPRGASESVTPKSSAGSSAGSTKSTITKTLKLRIVRPYNSAEVEKIVADEKNNREKIALEKNKDKVKEACSKHLKVAAYCTTQVERNACLFCKARKLDDKFYQKLRGQFPDAVFWQELGEILRQLQKQAAEIYNQSLIELYYEIFIKGRGFASASSVEHYLSDVCYTRAAELFKNAAIASGLRGKVKSNFRLKELKYMKSGLPTTKSDNFPIPLVKQKGGQYTGFEISSHNDDFIIKIPFGRWQVKKEIDKYRPWEKFDFEQVRKSPKPISLLLSTQRRKKNKGWSKDEGTEAEIRKVMNGDYQTSYIEVKRGSKTGEKSAWMLNLSIDVPKIDKGVDPSIIGGIDVGVKSPLVCAINNAFSRYSISDNELFHFNKKMFARRRILLKKNRHKRAGHGAKNKLKPISILTGKSERFRKKLIERWACEIADFFIKNKVGTVQMENLESMKRKEDSYFNIRLRGFWPYAEMQNKIEFKLKQYGIEIRKVAPNNTSKTCSKCGHLNNYFNFEYRKRNKFPHFKCEKCNFKENADYNAALNISNPKLKSTKEEP

SEQ ID NO: 1849 - protein, 726 aa, synthetic construct
SEVEFSHEYWMRHALTLAKRARDEREVPVGAILVLNNRVIGEGWNRAIGLHDPTAHAEIMALRQGGLVMQNYRLTDATLYVTFEPCVMCAGAMVHSRIGRVVFGVRNSKRGAAGSLMNVLNYPGVNHCVEITEGILVDECAALLCDFYRMPRQVLNAQKKAQSSISSGGSSGGCSGSEMPGASESVTPKSSGGSSAGSTKNAITKTLKLRIVRPYNSAEVEKIVADEKNNREKIALEKNKDKVKEACSKHLKVASYCTTQVERSACPFCKARKLDDKFYQKLGGQFPDAVFWQELGEILRQLQKQAAEIYNQSLIELYYEIFIKGRGFANASSVEHYLSNVCYTRAAELFKNAAIASGLRGKVKSNFRLKELKNMKSGLPTTKSDNFPIPLVKQKGGQYTGFEISSHNDDFIIKIPFGRWQEKKEINKYRPWEKFDFEQVRKSPKPISLLLSTQRRKRNKGWSKDEGTEAEIRKVMNGDYQTSYIEVKRGSKTGEKSAWMLNLSIDVPKIDKGVDPSIIGGIDVGVKSPLVCAINNAFSRYSISDNDLFRFNKKMFARRRILLKKNRHKRAGHGAKNKLKPISILTGKGERFRKKLIERWACEIADFFVKNKVGTVQMENLESMKRKEDSYFNIRLRGFWPYAEMQNKIEFKLKQYGIEIRKVAPNNTSRTCSKCGHLNNYFNFEYRKKNKFPHFKCEKCNFKEDADYNAALNISNPKLKSTKEEP

SEQ ID NO: 1850 - protein, 726 aa, synthetic construct
SEVEFSHEYWMRHALTLAKRARDEREVPVGAILVLNNRVIGEGWNRAIGLHDPTAHAEIMALRQGGLVMQNYRLIDATLYVTFEPCVMCAGAMIHSRIGRVVFGVRNSKHGAAGSLVNVLNYPGMNHRVEITEGILADECAALLCDFYRMPRQVFNARKKAQSSINPSGSSGGSSGSVTPGTSESATPESSGGGFGGSAKNTITKTLQLRIVRPYNSAEVEKIVADEKNNREKIALEKNKDKVKEACSKHLKVAPYCTTQVERNACLFCKARRLDDKFYQELRGQFPDAVFWQEIGEIFRQLQKQAAEIYNQSLVELYYEILIKGKGIANASSVEHYLSDVCYTRAAELFKNAAIASGLRNKIKSNFRLKELRNMKSGLPTTKSDNFPIPLVRQKGGQYTGFEISNHDGDFIIKIPFGRWQVKKEINKHRPWEKFDFEQVRKSPKPISLLLSTQRRKRNKGWSKDEGTEAEIRKVMNGDYQTSYIEVKRGSKIGEKSAWMLNLSIDVPKIDKGVDPSIIGGIDVGVKSPLVCAINNALSRYSISDNDLFHFNKKMFARRRILLRKNRHKRAGHGARNKLKPITVLTEKSERFRKKLIERWACEIANFFIKNKVGTVQMENLESMKRREDSYFNIRLRGFWPYAEMQSKIEFKLKQYGIKIRKVAPNNTSKTCSKCGHLNNYFNFEYRKKNKFPHFKCEKCNFKEDADYNAALNISNPKLKSTKEEP

SEQ ID NO: 1851 - protein, 726 aa, synthetic construct
SEVEFSHEYWMRHALTLAKRARDEREVPVGAVLVLNNRVIGEGWNRAIGLHDPTAHAEIMALRQGGLAMQNYRLVDATLYVTFEPCVLCAGAMVHSRIGRVVFGVRNSKRGAAGSLMNVLNHPGMSHRVEITGGILADECAALLCDFYRMPRQVFNAQKKARSNINSGGSSGGSSGSETLGTSESATPESSGGSSGGSAKNTITKTLKLRIVRPYNSTEVEKIVADEKDNREKIALEKNKDKVKEACSKHLKVASYCTTQVERNACLFCKARKLDDKFYQKLRGQFPDAVFWQELGEIFRQLQKQAAEIYNQSLIELYYEIFIKGKGFANASSVEHYLSDVCYTRAAELFKNAAIASGLRGKVKSNFRLKELKNMKSGLPTTKSDNFPIPLVKQKGGQYTGFEISSHNDDLIIKIPFGRWQVKKEIDKYRPWEKFDFEQVRKSPKPISLLLSTQRRKRNKGWSKDEGTEAEIRKVMNGDYQTSYIEVTRGSKIGEKSAWMLNLSIDVPKIDKGVDPSIIGGIDVGVKSPLVCAINNAFSRYSISDNDLFHFNKKMFARRRILLKKNRHKRAGHGAKNKLKPITILTEKSKRFRKKLIERWACEIADFFVKNKVGTVQMENLESMKRKEDSYFNIRLRGFWPYAEMQNKIEFKLKQYGIEIRKVAPNNTSKTCSKCGHLNNYFNFEYRKKNKFPHFKCEKCNFKENADYNAALNICNPKLKSTKEEP

SEQ ID NO: 1852 - protein, 726 aa, synthetic construct
SEVEFSHEYWMRHALTLAKRARDEREVPVGAVLVLNNRVIGEGWNRAIGLHDPTAHAEIMALHQGGLVMQNYRLIDATLYVTFEPCVMCAGAMIHSRIGRVVFGARNSKRGAAGSLMNVLSYPGMNHRVEITEGILADECAALLCDFYRMPRRVFNAQKKAQSSINSGGSSGGGSGSDTPGTSESPTPESSGGIPGGSAKNTITKTLKLRIVRPYNSAEVEKIVADEKNNREKIALEKNKDKVKEACSKHLKVAAYCTTQVERNACLFCKARKLDDKFYQKLRGQFPDAVFWQEIGEIFRQLQKQAAEIYNQSLIELYYEIFIKGKGFANASSVEHYLSDVCYTRAAELFKNAAIASGLRGKVKGNFRLKELKSMKSGLPTTKSDNFPIPLVKQKGGQYAGFEISSHNDDFIIKIPFGRWQVKKEIDKYRPWEKFDFEQVRKSPKPISLLLSTQRRKRNKGWSKDEGTEAEIRKVMNGDYQTSYIEVKRGSKTGEKSAWMLNLSIDVPKIDKGVDPSIIGGIDVGVKSPLVCAINNAFSRYSISDNDLFRFNKKMFARRRILLKKNRHKRAGHGAKNKLKPISILTGKGERFRKKLIERWACEIADFFIKNKVGTVQMENLESMKRKEDSYFNIRLRGFWPYAEMQNKIEFKLKQYGIKIRKVAPNNTSKTCSKCGHLNNYFNFEYRKKNKFPHFKCEKCNFKENADYNAALNISNPKLKSTKEEP

SEQ ID NO: 1853 - protein, 726 aa, synthetic construct
SEVEFSHEYWMRHALTLAKRARDEREVPVGAILVLNNRVIGEGWNRAIGLHDPTAHAEIMALRQGGLVMQNYRLVNATLYVTFEPCVMCAGAMIHSRIGRVVFGVRNSKRGAAGSLMNVLNYPGMNHRVEITEGILTDECAALLCDFYRMPHQVLNAQKKAQSSISSGGSSGGCSGSEMPGASESVTPKSSGGSSAGSTKNTITKTLKLRIVRPYNSAEVEKIVADEKSSREKIALERNKDKVKEACSEHLKVAAYCTTRVERNACLFCKARKLDDRFYQKLRGQFPDAVFWQETGEIFRQLQRQAAEIYNQSLIELYYEIFIRGRGFANASSVEHYLSDVCYTRAAELFKNAAIASGLRGKVKSNFRLKELKNMKSGLPTTKSDNFPIPLVKQKGGQYTGFEISNHNDDFIIKIPFGRWQVKKEIDKYRPWEKYDFEQVRKSPKPISLLLSTQRRKRSKGWSKDEGTEAEIRKVMNGDYQTSYIEVKRGSKTGEKSAWMLNLSIDVPKIDKGVDPSIIGGIDVGVKSPLVCAINNAYSRYSISDNDLFRFNKKMFARRRILLRKNRHKRAGHGAKNKLKPISILTGKSERFRKKLIERWACEIADFFIKNKVGTVQMENLESMKRKEDSYFNIRLRGFWPYAEMQNKIEFKLKQYGIEIRKVAPNNTSKTCSKCGHLNNYFNFEYRKKNKFPHFRCEKCNFKENADYNAALNISNPKLKSTKEEP

SEQ ID NO: 1854 - protein, 726 aa, synthetic construct
SEVEFSHEYWMRHALTLAKRARDEREVPVGAVLVLNNRVIGEGWNRAIGLHDPTAHAEIMALRQGGLVMQNYRLIDATLYVTFEPCVMCAGAMIHSRIGRVVFGVRNSKHGAAGSLVNVLNYPGMNHRVEVTEGILADECAALLCDFYRMPRQVFNARKKARSNINSGGSSGGSSGSETPGTCESATPESSGGSSSGSAKNTITKTLQLRIVRPYNSAEVEKIVADEKNNREKIALEKNKDKVKEACSKHLKVASYCTTQVERNACPFCKARKLDDKFYQKLRGQFPDAVFWQELGEILRQLQKQAAEIYNQSLIELYYEIFIKGRGFANAGSVEHYLSDVCYTRAAELFKNAAIASGLRGKVKSNFRLKELKNMKSGLPTTKSDNFPIPLVKQKGGQYTGFEISSHNDDFIIKIPFGRWQVKKEIDKYRPWEKFDFEQVRKSPRPISLLLSTQRRKRNKGWSKDEGTEAEIRKVMNGDYQTSYIEVKRGSKTGEKSAWMLNLSIDVPKIDKGVDPSIIGGIDVGVKSPLVCAINNAFSRYSISDNDLFRFNKKMFARRRILLKKNRHKRAGHGAKNKLKPISILTGKSERFRKKLIERWACEIADFFIKNKVGTVQMENLESMKRKEDSYFNIRLRGFWPYAEMQNKIEFKLEQYGIEIRKVAPNNTSKTCSKCGYLNNYFNFEYRKKNKFPHFKCEKCNFKENADYNAALNISNPKLKSTKEKP

SEQ ID NO: 1855 - protein, 726 aa, synthetic construct
SEVEFSHEYWMRHALTLAKRARDEREVPVGAVLVLNNRVIGGGWNRAIGLHDPTAHAEIMALRQGGLVMQNCRLVDATLYVTFEPCVMCAGAMIHSRIGRVVFGVRNSKRGAAGSLMNVLNYPGMNHCVEITEGILVDECAALLCDFYRMPRQVLNAQKKAQSSISSGGSSGGSSGSVTPGASGSVTPKSSGGSSAGSTKDTITKTLQLRIVRPYNSAEVEKIVADEKNNREKIALEKNKDKVKEACSKHLKVASYCTTQVERNACLFCKARKLDDKFYQKLRGQFPDAVFWQELGEILRQLQKQAAEIYNQSLIELYYEIFIKGRGFANASSVEHYLSDVCYTRAAELFKNAAIASGLRGKVKSNFRLKELKNMKSGLPTTKSDNFPIPLVKQKGGQYTGFEISSHNDDFIIKIPFGRWQAKKEIDKYRPWEKFDFEQVRKSPKPISLLLSTQRRKRNRGWSKDEGTEAEIRKVMNGDYQTSYIEVKRGSKIGEKSAWMLSLSIDVPKIDKGVDPSIIGGIDVGVKSPLVCAINNAFSRYSISDNDLFRFNKKMFARRRILLKKNRHKRAGHGAKNKLKPISILTGKSERFRKKLIERWACEIADFFIKNKVGTVQMENLESMKRKEDSYFNIRLRGFWPYAEMQNKIEFKLKQYGIEIRKVAPNNTSRTCSKCGHLNNYFNFEYRKKNKFPHFRCEKCNFKENADYNAALNISNPKLKSTKEGP

SEQ ID NO: 1856 - protein, 726 aa, synthetic construct
SEVEFSHEYWMRHALTLAKRARDEREVPVGAILVLNNRVIGEGWNRAIGLHDPTAHAEIMALRQGGLVTQNYRLIDATLYVTFEPCVMCAGAMIHSRIGRVVFGVRNSKHGAAGSLVNVLNYPGMNHRVEITEGVLADECAALLCDFYRMPRQVFNARKKAQSNINPGGSSGGSSGSETPGTSDSATPRSSGGSSGGSAKNTITKTLKLRIVRPYNSAEVEKIVADEKNNREKIALEKNKDKVKEACSKHLKVASYCTTQVERNACLFCKARKLDDKFYQKLRGQFPDAVFWQELGGIFRQLQKQAAEIYNQSLIELYYEIFIKGKGITNAGRVEHYLSDVCYTRAAELFKNAAIASGLRSKVRSNFRLKELKNMKSGLPTTKSDNFPIPLVKQKGGQYTGFEISSHNSDFIIKIPFGRWQVKKEIDKYRPWEKFNFEQVRKSPKPISLLLSTQRRKRNKGWSKDEGTEAEIRKVMNGDYQTSYIEVKRGSKTGEKSTWMLNLSIDVPKIDKGVDPSIIGGIDVGVKSPLVCAINNAFSRYSISDNDLFRFNKKMFARRRILLKKNRHKRAGHGAKNKLKPISILTGKSERFRKKLIERWACEIADFFIENKVGTVQMENLESMKRKEDSYFNIRLRGFWPYAEMQNKVEFKLKQYGIKVRKVAPNNTSKTCSKCGHLNNYFSFEYRKTNKFPHFKCEKCNFKENADYNAALNISNPKLKSTKEEP

SEQ ID NO: 1857 - protein, 726 aa, synthetic construct
SEVEFSHEYWMRHALTLAKRARDEREVPVGAILVLNNRVIGEGWNRAVGLHDPTAHAEIMALRQGGLVMQNYRLSDATLYVTFEPCVMCAGAMIHSRIGRVVFGVRNSKRGAAGSLMNVLNYPGMNHCVEITEGILVDECAALLCDFYRMPRQVLSAQKKAQSSVSSGGSSGGSSGSETPGASGSVTPKSSVGSSAGSTKNTITKTLKLRIVRPYNSAEVEKIVADEKNNREKIALEKNRDKVKEACSKHLKVVAYCTTQVERNACLFCKARKLDDKFYQRLRGQFPDAVFWQEIGEIFRQLQKQAAEIYNQSLIELYYEIFIKGRGFANAGSVEHYLSDVCYTRAAELFKNAAIASGLRGKVKSNFRLKELKNMKSGLPTTKSDNFPIPLVKQKGGQYTGFEISSHNDDFIIKIPFGRWQVKKEIDKYRPWEKFDFEQVRKSPKPISLLLSTQRRKRNKGWSKDEGTEAEIRKVMNGDYQTSYIEVKRGSKTGEKSAWMLNLSIDVPKIDKGVDPSIIGGIDVGVKSPLVCAINNAFGRYSISDNDLFRFNKKMFARRRILLKKNRHKRAGHGAKNKLKPISILTGKSERFRKKLIERWACEIADFFIKNKVGTVQMENLESMKRKEDSYFNIRLRGFWPYAEMQDKIEFKLKQYGIEIRKVAPNNTSKTCSRCGHLNNYFNFEYRRKNKFPHFKCEKCNFKEDADYNAALNISNPKQKSTREEP

SEQ ID NO: 1858 - protein, 726 aa, synthetic construct
SEVEFSHEYWMRHALTLAKRARDEREVPVGAILVLNNRVIGEGWNRAIGLHDPTAHAEIMALRQGGLVMQNYRLIDATLYVTFEPCVMCAGAMIHSRIGRVVFGVRNSKHGAAGSLVNVLNYPGMNHRVEITEGILADECAALLCDFYRMPRQVFSARRKAQSSISPGGSSGGSSGGETPGSSKSLTPESPGGSSGGSAKNTITKTLKLRIVRPYNSAEVEKIVADEKNNREKIALEKNKDKVREACSEHLKVAAYCTTQVERNACLFCKARRLDDKFYQKLRGQFPDAVFWQELGEIFRQLQKQAAVIYNQSLIELYYEIFIKGKGIANASRVEHYLSDVCYTRAAELFKNAAVASGLRGKVKSNFRLKELKNMKSGLPTTKSDNFPIPLVKQKGGQYTGFEISSHNDDFIIKIPFGRWQVRKEIDKYRPWEKYDFEQVRKSPKPISLLLSTQRRKRNKGWSKDEGTEAEIRKVMNGDYQTSYIEVKRGSKIGEKSAWMLNLSIDAPKIDKGVDPSIIGGIDVGVKSPLVCAINNAFSRYSISDNDLFHFNKKMFARRRILLKKNRHKRAGHGAKNKLKPISILTEKGERFRKKLIERWACEIADFFIKNKVGTVQMENLEGMKRKEDSYFNIRLRGFWPYAKMQSKIEFKLKQYGIEIRKVAPNNTSKTCSKCGHLNDYFNFEYRKKNKFPHFKCEKCNFKEDADYNAALNISNPKLKSTKEES

SEQ ID NO: 1859 - protein, 726 aa, synthetic construct
SEVEFSHEYWMRHALTLAKRARDEREVPVGAVLVLNNRVIGEGWNRAIGLHDPTAHAEIMALRQGGLVLQNYRLVDATLYVTFEPCVLCAGAMVHSRIGRVVFGARNSKRGAAGSLMNILNYPGMNHRVEITGGVLADECAALLCDFYRMPRQVFNAQKKVQSSINSGGSSGGSSGSETPSTSESATPESSGGSSGGSAKNTITKTLKLRIVRPYNSAEVEKIVADEKNSREKIALEKNKDKVKEACSRHLKVAAYCTTQVERNACLFCKARKLDDKFYQKLRGQFPDAVFWQEIGEIFRQLQKQAAEIYNQSLIELYYEIFIKGKGFANASSVEHYLSDVCYARAAELFKNAAIASGLRGKVKSNFRLKELKNMKSGLPTTKSDNFPIPLVKQKGGQYTGFEISSHNDDFIIKIPFGRWQVKKEIDKYRPWEKFDFEQVRKSPKPISLLLSTQRRKRNKGWSKDEGTEAEIRKVMNGDYQTSYIEVKRGSKIGEKSAWMLNLSIDVPKIDKGVDPSIIGGIDVGVKSPLVCAINNAFSRYSISDNDLFRFNKKMFARRRILLGKNRHKRAGHGVKNKLKPITILTEKSGRFRKKLIERWACEIADFFVKNKVGTVQMENLESMKRKEDSYFNIRLRGFWPYAEMQNKIEFKLKQYGIKVRKVAPNNTSKTCSKCGHLNNYFSFEYRKKNKFPHFKCEKCNFKENADYNAALNISNPKLKSTKEEP

SEQ ID NO: 1860 - protein, 726 aa, synthetic construct
SEVEFSHEYWMRHALTLAKRARDEREVPVGAVLVLNNRAIGEGWNRAIGLHDPTAHAEIMALRQGGLVMQNYRLIDATLYVTFEPCVMCAGAMVHSRIGRVVFGVRNSKRGAAGSLMNVLDYPGMGHRVEITEGILADECAALLCDFYCMPRQVFNAQKRAQSCINPGGSSGGSSGSGTPVTNESATPESSGGSSGGSAKNTITKTLKLRIVRPYNSAEVEKIVADEKDNRERIALEKNKGKVKEACSKHLKVAAYCTTQVERNACLFCKARKLDDKFYQKLRGQFPDAVLWQEIGEIFRQLQKQAAEIYNQSLIELYFEIFIKGKGFANASSVEHYLSDVCYTRAAELFKNAAIASGLRGKVKSNFRLKELKNMKSGLPTTKSDNFPIPLVKQKGGQYTGFEISSHNDDFIIKIPFGRWQVKKEIDKYRPWEKFDFEQVRKSPKPISLLLSTQRRKRNKGWSKDEGTEAEIRKVMNGDYQTSYIEVKRGSKIGEKSAWMLNLSIDVPKIDKGVDPSIIGGIDVGVRSPLVCAIDNAFSRYSISDNDLFHFNKKMFARRRILLKKNRHKRAGHGAKNKLKPISILTEKSKRFRKKLIERWACEIADFFVKNKVGTVQMENLESMKRKEDSYFNIRLRGLWPYAEMQNKIEFKLKQYGIEIRKVAPNNTSKTCSKCGHLNNYFNFEYRKKNKFPHFKCEKCNFKENADYNAALNISNPKLKSTKEEP

SEQ ID NO: 1861 - protein, 725 aa, synthetic construct
SEVEFSHEYWMRHALTLAKRARDEREVPVGAVLVLNNRVIGEGWNRAIGLHDPTAHAEIMALRQGGLVMQNYRLIDATLYVTFEPCVMCAGAMIHSRIGRVVFGVRNNKHGAAGSLVNVLNYPGMNHRVEITEGILADECAALLCDFYRMPRQVFNARKKGRSNINSGCSSGGSSGSETPGTSESATPESSGGSSGGSTKNTITKTLKLRIVRPYNSAEVEKIVADEKNNREIALEKNKDKVKEACSKHLKVAAYCTTQVERNACLFCRARRLDDKFYQKLRGQFPDAVFWQEIGEIFRQLQKQAAEIYNQSLVELYYEIFIKGKGIANASGVEHYLSDVCYTRAAELFKNAAIASGLRNKIKSNFRLKELRNMKSGLPTTKSDNFPIPLVRQKGGRYTGFEISNHNSDFIIKIPFGRWQVKKEIDKYRPWEKFDFAQVRKSPKPISLLLSTQRRKRNKGWSNDEGTEAEIRKVMNGDYQTSYIEVKRGSKIGEKSAWMLSLSIDVPKIDKGVDPSIVGGIDVGVKSPLVCAINNALGRFSISDNDLFHFNKKMFARRRILLRKNRHKRAGHGAKNKLKPISILTEKSKRFRKKLIERWACEIADFFIKNKVGTVQMEDLESMKRRGDSYFNIRLRGLWPYAEMQNKIEFKLKQYGIEIRKVAPNNTSKTCSKCGHLNNYFNFEYRKKNKFPHFKCEKCNFKENADYNAALNISNPKLKSTKEEP

SEQ ID NO: 1862 - protein, 726 aa, synthetic construct
SEVEFSHEYWMRHALTLAKRARDEREVPVGAILVLNNRVIGEGWNRTTGLHDPTAHAEIMALRQGGLVMQNHRLVDATLYVTFEPCVMCAGAMIHSRIGRVVFGVRNSKHGAAGSLMNVLNYPGMNHRVEITEGILADECAALLCDFYRMPRQVFNGRKKAQSSINSGGSSGGSSGSETPGTSENATPESSGGSSGGSAKNTITKTLQLRIVRPYNSAEVEKIVTDEKNNREKIALEKNKDKVKEACSKHLKIAAYCTTQVERNACLFCKARKLDDKFYQKLRGQFPDAVFWQELGEIFRQLQKQAAEIYNQSLIELYYEIFIKGKGFANASSVEHYLSDVCYTRAAELFKNAAIASGLRGKVKSNFRLRELKNMKSGLPTTKSDNFPIPLVKQKGGQYTGFEISSHNDDFIIKVPFGRWQAKKEIDKYRPWEKFDFEQVRKSPKPISLLLSTQRRKRNKGWSRDEGTEAEIRKVMNGDYQTSYIEVKRGSKTGEKSAWMLNLSIDVPKIDKGVDPSIIGGIDVGVKSPLVCAISNAFSRYSISDNDLFRFNKKMFARRRILLKKNRHKRAGHGAKNKLKPISILTGKSERFRKKLIERWACEIADFFIKNKVGTVQMENLESMKRKEDSYFNIRLRGFWPYAEMQNKIEFKLKQYGIEIRKVAPNNTSKTCSKCGHLNNYFNFEYRKKNKFPHFKCEKCNFKENADYNAALNISNPKLKSTKEEP

SEQ ID NO: 1863 - protein, 726 aa, synthetic construct
SEVEFSHEYWMRHALTLAKRARDKHEVPVGAVLVLNNRVIGEGWNRATGQNDPTAHAEIMALRQGGLVMQNHRLIDATLYVTFEPCVMCAGAMIHSRIGRVVIGVRNSRRGAAGSLMNVLNHPGMNHRVEITEGILADECAALLCDFYRMPRQVFNARKKAQSGINPSGSSGGSSGSVTPGTSESATPESSGGSSGGSAKNTITKTLKLRIVRPYNSTEVEKIVADEKNDREKIALEKNKDKVKEACSKHLKVASYCTTQVERNACLFCKARRLDDKFYQKLRGQFPDAVFWQEIGEIFRQLQKQAAEIYNQSLVELYYEIFIKGKGIVNASRVEHYLSDVCYTRAAELFKNAAIASGLRNKIKSNFRLKELRNMKSGLPTTKSDNFPIPLVKQKGGQYTGFEISSHNDDFIIKIPFGRWQVRKEIDKYRPWEKFNFEQVRKSPKPISLLLSTQRRKRNKGWSKDEGTEAEIRRVMNGDYQTSYIEVKRGSKIGEKSAWMLNLSIDVPKIDKGVDPSIIGGIDVGVKSPLVCAINNAFSRYSISDNDLFHFNKKMFARRRILLKKNRHRRAGHGAKNKLKPITILTEKSVRFRKKLIERWACEIADFFIKNKVGTVQMENLESMKRKEDSYFNIRLRGFWPYAEMQNKIEFKLKQYGIEIRRVAPNNTSRTCSKCGHLNNYFNFEYRRKNKFPHFKCEKCNFKEDADYNAALNISNPKLKSTKEEP

SEQ ID NO: 1864 - protein, 726 aa, synthetic construct
SEVEFSHEYWMRHALTLAKRARDEREVPVGAILVLNNRVIGEGWNRAIGLHDPTAHAEIMALRQGGLVMQNYRLIDATLYVTFEPCVMCAGAMIHSRIGRVVFGVRNNKHGAAGSLVNVLNYPGMNHRVEITEGILADECAALLCDFYRMPRQVFNARKKAQSSINPGGSSGGSSGSETPGTSESATPESSGGSSGSSAKNTITKTLKLRIVRPYNSAEVERIVADEKNNREKIALEKNKDKVKEACSKHLKMASYCTTQVERNACLFCKARKLDDKFYQKLRDQFPDAMFWQEIGEIFRQLQRQAAEIYNQSLIELYYEVFIKGKGFANASSVEHYLSDVCYTRAAELFKNAAIASGLRGKVKSNFRLKELKNMRSGLPTTKSDNFPIPLVKQKGGQYTGFEISDHNSDFIIKIPFGRWQAKKEIDKYRPWEKFDFEQVRKSPKPISLLLSTQRRKKNRGWSKDEGTEAEIKKVMNGDYQTSYIEVKRGSKIGEKSAWMLNLSIDVPKIDKGVDPSIIGGIDVGVKSPLVCAIDNAFSRYSISDNDLYHFNKKMFAKRRILLKKNRHKRAGHGAKNKLKPISILTEKSERFRKKLIERWACEIADFFIKNKVGTVQMENLESMKRREDSYFNTRLRGFWPYAEMQNKIEFKLKQYGIKIRKVAPNNTSKTCSKCGHLNNYFNFEFRKKNKFPHFKCEKCNFKENADYNAALNISNPKLKSTKEEL

SEQ ID NO: 1865 - protein, 726 aa, synthetic construct
SEVEFSHEYWMRHALTLAKRARDEREVPVGAVLVLNNRVIGVGWNRAIGLHDPTAHAEIMALRQGGLVMQNYRLIDATLYVTFEPCAMCAGAMIHSRIGRVVFGVRNSKHGAAGSLVNVLNYPGMNHRVEITEGILADECAALLCDFYRMPRQVFNARKKAQSSINPGGSSGGSGGSETPGTSESATPESSGGSSGGSAKNTITKTLKLRIVRPYNSAEVEKIVADEKNNREKIALEKNKDKVKEACSKHLKVAPYCTTQVERNACPFCKARKLDDKFYQKLRGQFPDAVFWQELGEILRQLQKQAAEIYNQSLIELYYEIFVKGKGFANASSVEHYLSDVCYTRAAELFKNAAIASGLRGKVKSNFRLKELKNMKSGLPTTKSDNFPIPLVKQKGGQYTGFEISSHNDDFIIKIPFGRWQVKEEIDKYRPWEKFDFEQVRRSPKPISLLLSTQRRKKNKGWSKDEGTEAEIRRVMNGDYQTSYIEVKRGSKIGEKSAWMLNLSIDVPKIDKGVDPSIIGGIDVGVKSPLVCAINNSSSRYSICDNDLFRFNKKMFARRRILLKKNGHKRAGHGAKNKLKPITIMTEKSKRFRKKLIERWACEIADFFIKNKVGTVQMENLESMKRKEDSYFNIRLRGFWPYAEMQNKIEFKLKQYGIEIRKVAPNNTSKTCSECGHLNNYFNFEYRKKNKFPHFKCEKCNFKEDADYNAALNISNPKLKSTKEEP

SEQ ID NO: 1866 - protein, 726 aa, synthetic construct
SEVEFSHEYWMRRALTLAKRARDEREVPVGAVLVLNNRVIGVGWNRAVGLHDPTAHAEIMALRQGGLVMQNYRLIEATLYVTFEPCIMCAGAMIHSRIGRVVFGVRNSKRGAAGSLMNVLNYPGMNHRVEITEGILADECAALLCDYYRMPRQVFNARKKAQSSINSGGSSDGGSGSETPGTSESATPESSGGSSGGSAKNTITKTLKLRIVRPYNSAEVEKIVADEKNNREKIALEKNKDKVKEACSEHLKVAAYCTTQVERSACLFCKARKLDDKFYQKLRGQFPDAVFWQEIGEIFRQLQKQAAEIYNQSLIELYYEIFVKGKGFANASSVEHYLSDVCYTRAAELFKNAAIASGLRGKVKSNFRLKELKNMKSGLPTTKSDNFPIPLVKQKGGQYAGFEISSHNDDFIIKIPFGRWQAKKEIDKYRPWEKFDFEQVRKSPKPISLLLSTQRRKRNKGWSKDEGTEAEIRKVMNGDYQTSYIEVKRGNKTGEKSAWMLNLSIDVPKIDKGVDPSIIGGIDVGVKSPLVCAVNNAFSRYSICDNDLFRFNKKMFARRRILLKKNRHKRAGHGAKNKLKPITILTKKSERFRKKLIERWVCEVADFFIKNKVGTVQMENLESMKRKEDSYFNIRLRGFWPYAEMQNKIEFKLKQYGIKIRKVAPNNTSRTCSKCGHLNNYFSFEYRKKNKFPHFKCEKCNFKEDADYNAALNISNPKLKGTKEEL

SEQ ID NO: 1867 - protein, 726 aa, synthetic construct
SEVEFSHEYWMRHALTLAKRARDEREVPVGAVLVLNNRVIGEGWNRAIGLHDPTAHAEIMALRQGGLVMQNYRLIDATLYVTFEPCVMCAGAMIHSRIGRVVFGVRNNKRGAAGSLMNVLNYPGMNHRVEITEGILADECAALLCDFYRMPRQVLNAQKKAQSSINSGGSSGGSSGSETPGASESVTPKSSGGSSGGSAKNTITKTLKLRIVRPYNSAEVEKIVADEKNNREKIALEKNRGKVKEACSKHLEVAAYCTTQVERNACLFCKARKLDDKFYQKLRGQFPDAVFWQELGEIFRQLQKQAAEIYNQSLIELYYEIFIKGKGFANASSVEHYLSDVCYTRAAELFKNAAIASGLRGKVKSNFRLRELKNMKSGLPTTKSDNFPIPLVRQKGGQYTGFEISSHNDDFIIKIPFGRWQVRKEIDKYRPWEKFDFEQVRKSPKPISLLLSTQRRKRNKGWSKDEGTEAEIRKVMNGDYQTSYIEVKRGSKTGEKSAWMLNLSIDVPKIDKGVDPSVIGGIDVGVKSPLVCAINNAFSRYSISDNDLFHFNKKMFARRRILLKKNGRKRVGHGAKNKLKPITILTEKSKRFRKKLIERWACEIAGFFIKNKVGTVQMENLESMKRKEDSYFNIRLRGFWPYAEMQNKIEFKLKQYGIEIRKVAPDNTSKTCSMCGHLNNYFNFEYRKKNKFPHFKCEKCNFKEDADYNAALNISNPKLKSTKEEP

SEQ ID NO: 1868 - protein, 726 aa, synthetic construct
SEVEFSHEYWMRHALSLAKRARDEREVPVGAVLVLNNRIIGEGWNRAIGLHDPTAHAEIMALRQGGLVMQNYRLTDATLYVTFEPCVMCAGAMVHGRIGRVVFGVRNSKRGAAGSLMNVLNYPGVNHCVEITEGILADECAALLCDFYRMPRQVFNARKRAQSSINPGGSSGGCSGSEMPGASESVTPKSSGGGSSGSAKNTFTKTLQLRIVRPYNSAEVEKIVADEKDNREKIALEKNKDKVREACSRHLKVASYCTTQVERNACPFCKARKLDDKFYQKLRGQFPDAVFWQELGEILRQLQKQAAEIYNQSLIELYYEIFIKGRGFANASSVEHYLSDVCYTRAAELFKNAAIASGLRGKVKSNFRLKELKNMKSGLPTTKSDNFPIPLVKQKGGQYTGFEISSHNDDFIIKIPFGRWQVKKEIDKYRPWEKFDFEQVRKSPKPISLLLSTQRRKRNKGWSKDEGTEAEIRKVMNGDYQTSYIEVKRGSKIGEKSAWMLNLSIDVPKIDKGVDPSIIGGIDVGVKSPLVCAINNASSRYSISDNDLFHFNKKMFARRRILLKKNGRKRAGHGAKNKLKPITIMTEKSGRFRKKLIERWACEIADFFIKNKVGTVQMENLESMRRREDSYFNIRLRGFWPYAEMQNKIEFKLKQYGIKIRKVAPNNTSKTCSKCGHLNGYFNFEYRKRNKFPRFKCEKCNFKEDADYNAALNISNPKLKSTKEEP

SEQ ID NO: 1869 - protein, 726 aa, synthetic construct
SEVEFSHEYWMRHALTLAKRARDEREVPVGAILVLNNRVIGEGWNRAIGLHDPTAHAEIMALRQGGLVMQNYRLIDATLYVTFEPCVMCAGAMILSRIGRVVFGVRNNKHGAAGSLVNVLDYPGMNHRVEITEGILADECAALLCDFYRMPRQVFNARKKAQSSISPGGSSGGSSGSETPGTSESATPESSGGSSGDSAKNTITKTLKLRIVRPYNSAEVEKIVADEKNNREKIALEKNKDKVKEACSKHLKVAAYCTTQVERNACLFCKARKLDDKFYQKLRGQFPDAVFWQEIGEVFRQLQKQAAEIYNQSLIELYYEIFIKGKGFANASSVEHYLSDVCYTRAAELFKNAAIASGLRGKVKSNFRLKELKNMKSGLPTTKSDNFPIPLVKQKGGQYTGFEISSHNDDFIIKIPFGRWQVKKEINKFRPWEKFDFEQVRKSPKPISLLLSTQRRKRNKGWSRDEGTEAEIRKVMNGDYQTSYIEVKRGSKIGEKSAWMLNLSIDVPKIDKGVDPSIIGGIDVGVKSPLVCAINNAFSRYSISDNDLFHFNKKMFARRRILLKKTRHKRAGHGAKNKLKPISILTEKSERFRKKLIERWACEIADFFIKNKVGTVQMENLESMKRREDSYFNIRLRGFWPYAKMQNKIEFKLKQYGIKIRKVAPNNTSKTCSKCGHLNNHFNFEYRKKNKFPHFKCEKCNFKENADYNAALNISNPKLKSTKGEP

SEQ ID NO: 1870 - protein, 726 aa, synthetic construct
SEVEFSHEYWMRHALTLAKRARDEREVPVGAILVLNNRVIGEGWNRAIGLHDPTAHAEIMALRQGGLVMQNYRLIDATLYVTFEPCVMCAGAMIHSRIGRVVFGVRNSKHGAAGSLVNVLNYPGMNHRVEITEGILADECAALLCDFYRMPRQVFNARKKAQSSINSGGSSGGGSGSDTPSTSESTTPESSGGSSGGPAKSTITKTLKLRIVRPYNSAEVEKIVADEKNNREKIALEKNKDKVKEACSEHLKVAAYCTTQVERSACLFCKARKLDDKFYQKLRGQFPDAVFWQEIGEIFRQLQKQAAEIYNQSLIELYYEIFIKGKGFANASSVEHYLSDVCYTRAAELFKNAAIASGLRGKVKSNFRLKELKNMKSGLPTTKSDNFPIPLVKQKGGQYTGFEISSHNDDFIIKIPFGRWQVKKEIDKYRPWEKFDFEQVRKSPKPISLLLSTQRRKRNKGWSKDEGTEAEIRKVMNGDYQTSYIEVKRGSKIGEKSAWMLNLSIDVPKIDKGVDPSIIGGIDVGVRSPLVCAINNAFSRYSISDNDLFHFNKKMFARRRILLKKNGHKRAGHGAKNKLKPITIMTEKSKRFRRKLIERWACEIADFFIKNKVGTVQMENLESMKRKEDSYFNVRLRGFWPYAEMQNKIEFKLKQYGIEVRKVAPNNTSKTCSRCGHLNNYFNFEYRRKNKFPHFKCEKCNFKENADYNAALNISDPKLKSTKEEP

SEQ ID NO: 1871 - protein, 726 aa, synthetic construct
SEVEFSHEYWMRHALTLAKRARDEREVPVGAVLVLNNRVIGVGWNRAIGLHDPTAHAEIMALRQGGLVMQNYRLTDATLYVTFEPCVMCAGAMVHSRIGRVVFGVRNSKRGAAGSLMNVLNYPGMSHCVEITEGILVDECAALLCDFYRMPRQVLNAQKKAQSSISSGGSSGGSGGGETPGASESVTPKSSGGSSAGSTKNTITKTLKLRIVRPYNSAEVEKIVADEKNNREKIALEKNKDKVKEACGKHLKVAAYCTTQVERNACLFCKARKLDDKFYQKLRGQFPDAVFWQEIGEIFRQLQKQAAETYNQSLIELYYEIFIKGKGFANASSVEHYLSDVCYTRAAELFKNAAIASGLRGKVKSNFRLKELKNMKSGLPTTKSDNFPIPLVRQKGGQYTGFEVSSHNDDFIIKIPFGRWQVKKEIDKYRPWEKFDFEQVRKSPRPISLLLSTQRRKRNKGWSKDEGTEAEIRKVMNGDYQTSYIEVKRGSKIGEKNVWMLNLSIDVPKIDKGVDPSIIGGIDVGVKSPLVCAINNAFNRYSISDNNLFHFNKKMFARRRILLKKNRHKRAGHGAKNKLKPISILTEKSERFRKKLIERWACEIADFFIRNKVGTVQMENLEGMKRKEDSYFNIRLRGFWPYAEMQNKIEFKLKQYGIKIRKVAPNNTSKTCSKCGHLNNYFSFEYRKKNKFPHFKCEKCNFKENADYNAALNISNPKLKSTKEEP

SEQ ID NO: 1872 - protein, 726 aa, synthetic construct
SEVEFSHEYWMRRALTLAKRARDEREVPVGAILVLNNRVIGEGWNRAIGLHDPTAHAEIMALRQGGLVMQNYRLIDATLYVTFEPCVMCAGAMIHSRIGRVVFGVRNNKHGAAGSLVNVLNHPGMNHRVEITEGILADECAALLCDFYRMPRQVFNARKKAQSSINSGGSSGGSSGSETPGTSESATPESSGGGSSGSAKNTITKTLQLRIVRPYNSAEVEEIVADEKNNREKVALEKNKDKVKEACSEHLKVAAYCTTQVERNACLFCKARRLDDKFYQKLRGQFPDAVFWQEIGEIFRQLQKQAAETYNQSLIELYYEIFIKGKGIANASNVEHYLSDVCYTRAAELFKNAAIASGLRNKIKSNFRLKELRNMKSGLPTTKSDNFPIPLVKQKGGQYTGFEISNHNGDFIIKIPFGRWQAKKEIDKYRPWEKFDFEQVRKSPKPISLLLSTQRRKRNRGWSKDEGTEAEIKRVMNGDYQTSYIEVKRGSKVGEKSAWMLNLSIDVPKIDKGVDPSIIGGIDVGVKSPLVCAINNAFSRYSISDNDLFHFNKKMFARRRILLRKNRHKRAGHGAKNKLKPITMMTEKSKRFRKKLIERWACEIADFFIKNKVGTVQMENLESMKRKEDSYFNIRLRGFWPYAEMQDKIEFKLKQYGIVVRKVAPNNTSKTCSKCGHLNHYFNFEYRKKNKFPHFKCEKCNFKEDADYNAALNISNPKLESTKGEP

SEQ ID NO: 1873 - protein, 726 aa, synthetic construct
SEVEFSHEYWMRRALTLAKRARDEREVPVGAVLVLNNRAIGVGWNRAVGLHDPTAHAEIMALRQGGLVMQNYRLTDATLYVTFEPCVMCAGAMIHSRIGRVVFGVRNSKRGAAGSLMNVLNYPGMNHCVEITEGILVDECAALLCDFYRMPRQVLNAQKKAQSSISSGGSSGGSSCSETPGASESVTPKSSGGSSAGSTKDAITKTLKLRIVRPYNSAEVEKIVADEKNNREKIAMEKNKDKVKEACSKHLKVASYCTTQVERNACLFCKARKLDDKFYQKLRGQFPDAVFWQELGGIFRQLQKQAAEIYNQSLIELYYEIFIKGKGITNASRVEHYLSDVCYTRAAELFKNAAIASGLRGKVKSNFRLKELKNMKSGLPTTKSDNFPIPLVKQKGGQYTGFEISSHNDDFIIKIPFGRWQVRKEIDKYRPWEKFDFEQVRKSPKPISLLLSTQRRKRNKGWSKDEGTEAEIRKVMNGDYQTSYIEVKRGSKTGEKSTWMLNLSIDVPKIDKGVDPSIIGGIDVGVKSPLVCAINNAFSRYSISDNDLFRFNKKMFARRRILLKRNRHKRAGHGAKNKLKPISILTGKSERFRKKLIERWACEIADFFIKNKVGTVQMENLESMKRKEDSYFNIRLRGFWPYAEMQNKIEFKLKQYGIEIRKVAPNNTSKTCSKCGHLNNYFNFEYRKKNKFPHFKCEKCNFKEDADYNAALNISNPKLKSTKEEP

SEQ ID NO: 1874 - protein, 726 aa, synthetic construct
SEVEFSHEYWMRHALTLAKRARDEREVPVGAVLVLNNRVIGEGWNRAIGLHDPTAHAEIMALRQGGLVLQNYRLVDATLYVTFEPCVMCAGAMIHSRIGRVVFGIRNSKRGAAGSLTNVLNHPGMSHRVEVTEGILADECAALLCDFYRMPRRVFNAQKKAQSTINSGGSSGGSSGSETPGTSESPTPESSGGSPGGSAKNTITKTLKLRIVRPYNSAEVEKIVADEKNNREKIALEKNKDKVKEACSKHLKVAAYCTTQVERNACLFCKARKLDDKFYQKLRGQFPDAVFWQELGEIFRQLQKQAAEIYNQSLIELYYKIFIKGKGFANASSVEHYLSDVCYTRAAELFKNAAIASGLRGKVKSNFRLKELKNMKSGLPTTKSDNFPVPLVKQKGGQYTGFEISSHNDDFIIKIPFGRWQVKKEIDKYRPWEKFDFEQVRKSPKPISLLLSTQRRKRNKGWSKDEGTEAEIRKVMNGDYQTSYIEVKRGSKTGEKSAWMLNLSIDVPKIDKGVDPSIIGGIDVGVKSPLVCAINNAFSRYSISDNDLFRFNKKMFARRRILLKKNRHKRAGHGAKNKLKPISILTGKSERFRRKLIERWACEIADFFIKNKVGTVQMENLESMKRKEDSYFNIRLRGFWPYAEMQNKIEFKLKQYGIEIRKVAPDNTSKTCSKCGHLNNYFNFEYRKKNKFPHFKCEKCNFKENADYNAALNISNPKLKSTKEEP

SEQ ID NO: 1875 - protein, 726 aa, synthetic construct
SEVEFSHEYWMRHALTLARRARDEREVPVGAILVLNNRVIGEGWNRAIGLHDPTAHAEIMALRQGGLVMQNYRLVDATLYVTFEPCVMCAGAMIHSRIGRVVFGVRNSKRGAAGSLMNVLNYPGMNHCVEITEGILVDECAALLCDFYRMPRQVLNAQKKAQPSISFGGSSGGSSGSGTPGASESATPESSGGSSGGSAKNTITKTLQLRIVRPYNGAEVEKIVTDEKNNREKIALEKNKDKVKEACSKHLKVASYCTTQVERNACLFCKARKLDDKFYQKLRGQFPDAVFWQELGGIFRQLQKQAAEIYNQSLIELYYEIFIKGKGITNASRVEHYLSDVCYTRAAELFKNAAIASGLRSKVRSNFRLKELKNMKSGLPTTKSDNFPIPLVKQKGGQYTGFEISSHNSDFIIKIPFGRWQEKEEIDKYRPWEKFDFEQVRKSPKPISLLLSTQRRKKNKGWSKDEGTEAEIRRVMNGDYQTSYIEVKRGSKIGEKSAWMLNLSIDVPKIDKGVDPSIIGGIDVGVKSPLVCAINNAFSRYSISDNDLFHFNKKMFARRRILLKKNRHRRAGHGAKNKLKPITILTEKSVRFRKKLIERWACEIADFFIKNKVGTVQMENLESMKRKEDSYFNIRLRGFWPYAEMQNKIEFKLKQYGIKIRKVAPNNTSRTCSKCGHLNNYFSFEYRKKNKFPHFKCEKCNFKEDADYNAALNISNPKLKGTKEEL

SEQ ID NO: 1876 - protein, 726 aa, synthetic construct
SEVEFSHEYWMRHALTLAKRARDEREVPVGAILVLNNRVIGEGWNRAIGLHDPTAHAEIMALRQGGLVLQNYRLVDATLYVTFEPCVLCAGAMVHSRIGRVVFGARNSKRGAAGSLMNILNYPGMNHRVEITEGILADECAALLCDFYRMPRQVFNAQKKAQSSINSGGSSGGSSGSETPSTSESATPESSGGSSGGSAKNTITKTLKLRIVRPYNSAEVEKIVADEKNNREKIALERNRDKVKEACSEHLRVAAYCTTQVERNACLFCKARKLDDKFYQKLRGQFPDAVFWQEIGEIFRQLQKQAAEIYNQSLVELYYEIFIKGKGITNASRVEHYLSDVCYTRAAELFKNAAIASGLRSKVRSNFRLKELKNMKSGLPTTKSDNFPIPLVKQKGGQYTGFEISSHNSDFIIKIPFGRWQVKEEIDKYRPWEKFDFEQVRKSPKPISLLLSTQRRKKNKGWSKDEGTEAEIRRVMNGDYQTSYIEVKRGSKIGEKSAWMLNLSIDVPKIDKGVNPSIIGGIDVGVKSPLVCAINNSSSRYSISDNDLFRFNKKMFARRRILLGKNRHKRAGHGVKNKLKPITILTEKSGRFRKKLIERWACEIADFFIKNKVGTVQMENLESMKRKEDSYFNIRLRGFWPYAEMQNKIEFKLKQYGIEIRKVAPNNTSKTCSKCGHLNNYFNFEYRKKNKFPHFKCEKCNFKENADYNAALNISNPKLKSTKEEP

SEQ ID NO: 1877 - protein, 726 aa, synthetic construct; identical to SEQ ID NO: 684

SEQ ID NO: 1878 - protein, 726 aa, synthetic construct
SEVEFSHEYWMRHALTLAKRARDEREVPVGAVLVLNNRVIGEGWNRAIGLHDPTAHAEIMALRQGGLAMRNYRLVDATLYVTFEPCVLCAGAMVHSRIGRVVFGVRNSKRGAAGSLMNVLNHPGMNHRVEITGGILADECAALLCDFYRMPRQVFNAQKKARSNINSGGSSGGSSGSETPGTSESATPESSGGSSGGSAKNTITKTLKLRIVRPYNSAEVEKIVADEKNDREKIALEKNKDKVKEACSEHLKVAAYCTTQVERSACLFCKARKLDDKFYQKLRGQFPDAVFWQEIGEIFRQLQRQAAEIYNQSLIELYYEILIKGKGFANASSVEHYLSDVCYARAAELFKNAAIASGLRGKVKSNFRLKELKNMRSGLPTTKSDNFPIPLVKQKGGQYAGFEISSHNDDFIIKIPFGRWQVKKEIDKYRPWEKFDFEQVRKSPKPISLLLSTRRRKRNKGWSRDEGTEAEIRKVMNGDYQTSYIEVKRGSKIGEKSAWMLSLSIDVPKIDKGVDPSIIGGIDVGVKSPLVCAINNAFCRYSISDNDLFHFNKKMFARRRILLKKSRHKRAGHGAKNKLKPISILTEKSKRFRKKLIERWACEIADFFIKNKVGTVQMENLESMKRKEDSYFNIRLRGFWPYAEMQNKIEFKLKQYGIEIRKVAPNNTSKTCSKCGHLNNYFNFEYRKKNKFPHFKCEKCNFKENADYNAALNISNPKLKSTKEEP

SEQ ID NO: 1879 - protein, 726 aa, synthetic construct
SEVEFSHEYWMRHALTLAKRARDEREVPVGAVLVLDNRVIGVGWNRAIGLHDPTAHAEIMALRQGGLVMQNYRLTDATLYVTFEPCVMCAGAMVHSRIGRVVFGVRNSKRGAAGSLMNVLNYPGMSHCVEITEGILADECAALLCDFYRMPRQVFNARKKAQSSINPGGSSGGSSGSETPGTSESATPKSSGGSSGGSAKNTITKALQLRIVRPYNSAEVEKIVADEKNNREKIALEKNKDKVKEACSKHLKVASYCTTQVERNACPFCKARKLDDKFYQKLRGQFPDAVFWQEIGEIFRQLQKQAAEIYNQSLIELYYEIFIKGKGFANASSVEHYLSDVCYTRAAELFKNAAIASGLRGKVKSNFRLRELKNMKSGLPTTKSDNFPIPLVKQKGGQYTGFEISSHNDDFIIKIPFGRWQVKEEIDKYRPWEKFDFEQVRKNPKPISLLLSTQRRKRNKGWSKDEGTEAEIRRVMNGDYQTSYIEVKRGSKIGEKSTWMLNLSIDVPKIDKGVDPSIIGGIDVGVKSPLVCAINNAFSRYSISDNDLFRFNKKMFARRRILLKKNRHKRAGHGAKNKLKPISILTGKSERFRKKLIERWACEIADFFIKNKVGTVQMENLESMKRREDSYFNIRLRGFWPYAEMQNKIEFKLKQYGIEIRKVAPNNTSKTCSRCGHLNNYFNFEHRKKNKFPRFKCEKCNFKENADYNAALNISNPKLKSTKEEP

SEQ ID NO: 1880 - protein, 726 aa, synthetic construct
SEVEFSHEYWMRHALTLAKRARDEREVPVGAILVLNNRVIGEGWNRAIGLHDPTAHAEIMALRQGGLVMQNYRLIDATLYVTFEPCVMCAGAMIHSRIGRVVFGVRNNKHGAAGSLVNVLNYPGMNHRVEITEGILADECAALLCDFYRMPRQVFNARKKAQSSINPGGSSGGSSGSETPGTSESATPESSGGSSGSSAKNTITKTLKLRIVRPYNSAEVEKIVADEKNNREKIALEKNKDKVKEACSKHLKVAAYCTTQVERNACLFCKARRLDDKFYQKLRGQFPDAVFWQEIGEIFRQLQKQAAEIYNQSLIELYYEIFIKGKGFANASSVEHYLSDVCYTRAAGLFKNAAIASGLRGKVKSNFRLKELKNMKSGLPTTKSDNFPIPLVKQKGGQYTGFEISSHNDDLIIKIPFGRWQVKKEIDKYRPWEKFDFEQVRKSPKPISLLLSTRGRKRNKGWSKDEGTEAEIRKVMNGDYQTSYIEVKRGSKIGEKSAWMLNLSIDVPKIDKGVDPSIIGGIDVGVKSPLVCAINNAFSRYSISDNELFHFNKKMFARRRILLKKNRHKRAGHGAKNKLKPISVLTEKSGRFRKKLIERWACEIADFFIKNKVGTVQMENLGSMKRKEDSYFNVRLRGFWPYAEMQNKIEFKLKQYGIEIRKVAPDNTSKTCSKCGHLNNYFNFEYRKKNKFPHFKCEKCNFKEDADYNAALNISNPKLKSTKEEP

SEQ ID NO: 1881 - protein, 726 aa, synthetic construct
SEVEFSHEYWMRHALTLAKRARDEREVPVGAVLVLNNRVIGEGWNRAIGLHDPTAHAEIMALRQGGLVMQNYRLIDATLYVTFEPCAMCAGAMVHSRIGRVVFGVRNSKRGAAGSLMNVLNYPGMDHRVEITGGILADECAALLCDFYRMPRQVFNARRKAQSSINPGGSSGGRSGSETPGTSESATPESSGGSSGGSAKNTITKTLKLRIVRPYNSAEVEKIVTDEKNNREKIALEKNKDKVKEACSKHLKVAAYCTTQVERNACLFCKARKLDDKFYRKLRGQFPDAVFWQEIGEIFRQLQKQAAEIYNQSLIELYYEIFIKGKGFANASSVEHYLSDVCYTRAAELFKNAAIASGLRGKVKSNFRLKELKNMKSGLPTTKSDNFPVPLVKQKGGQYTGFEISNHNSDFIIKIPFGRWQVKKEINKYRPWEKFDFEQVRKSPKPISLLLSTQRRKRNRGWSKDEGTEAEIRKVMNGDYQTSYIEVKRGSKIGEKSAWMLNLSIDVPRIDKGVDPSIIGGIDVGVKSPLVCAINNAFSRYSISDNDLFHFNKKMFARRRILLKKNRHKRAGHGAKNKLKPITILTEKSGRFRKKLIERWACEIADFFIKNKVGTVQMENLEGMKRKEDSYFNIRLRGFWPYAEMQNKIEFKLKQYGIEIRKVAPNNTSKTCSKCGHLNNYFNFEYRKKNKFPHFKCEKCNFKENADYNAALNISNPKLKSTKEEP

SEQ ID NO: 1882 - protein, 726 aa, synthetic construct
SEVEFSHEYWMRHALTLAKRARDGREVPVGAVLVLNNRVIGEGWNRAIGLHDPTAHAEIMALRQGGLVMQNYRLTDATLYVTFEPCVMCAGAMIHSRIGRVVFGVRNSKRGAAGSLMNVLNYPGMNHCVEITEGILVDECAALLCDFYRMPRQVLSAQKKAQSSVSSGGSSGGSSGSETPGASGSVTPKSSVGSSAGSTKNTITKTLKLRIVRPYNSAEVEKIVADEKNNREKIALEKNKGKVKEACSKHLKVASYCTTQVERNACPFCKARKLDDKFYQKLRGQFPDAVFWQELGGILRQLQKQAAEIYNQSLIELYYEIFIKGRGFANASSVEHYLSDVCYTRAAELFKNAAIASGLRGKVKSSFRLKELKNMKSGLPTTKSDNFPIPLVKQKGGQYTGFEISSHNDDFIIKIPFGRWQVKKEIDKYRPWEKFDFEQVRKSPKPISLLLSTQRRKRNKGWSKDEGTEAEIRKVMNGDYQTSYIEVKRGSKIGEKSAWMLNLSIDVPKIDKGVDPSIIGGIDVGVKSPLVCAINNALSRYSISDNDLFHFNKKMFARRRILLRKNRHKRAGHGAKNKLKPITIMTEKSKRFRKKLIERWACEIADFFTKNKVGTVQMENLESMKRREDSYFNIRLRGFWPYAEMQNKIEFKLKQYGIEIRKVTPNNTSKTCSRCGHLNNYFNFEYRKKNKFPHFKCEKCNFKENADYNAALNISNPKLKSSKEEP

SEQ ID NO: 1883 - protein, 726 aa, synthetic construct
SEVEFSHEYWMRHALSLAKRARDEREVPVGAVLVLNNRIIGEGWNRAIGQHDPTAHAEIMALRQGGLVMQNYRLTDATLYVTFEPCVMCAGAMIHSRIGRVVFGVRNSKRGAAGSLTNVLNYPGMNHRVEITEGILVDECAALLCDFYRMPRQVFNAQKKAQSTINSGGSSGGSSGSETPGTSESPTPESSGGSPGSSAKNTITKTLKLRIVRPYNSAEVEKIVAEEKNNREKIALEKNKDKVKEACSKHLKVAAYCTTQVERNACLFCKARRLDDKFYQKLRGQFPDAVFWQEIGEIFRQLQKQAAEIYNQSLIELYYEIFIKGKGFANASSVEHYLSDVCYTRAAELFKNAAIASGLRGKVKSNFRLKELKNMKSGLPTTKSDNFPIPLVKQKGGQYTGFEISSHNDDFIIKIPFGRWQVKKEIDKYRPWEKFDFEQVRKSPKPISLLLSTQRRKRNKGWSKDEGTEAEIRKVMNGDYQTSYIEVKRGSKTGEKSAWMLNLSIDVPKIDKGVDPSIIGGIDVGVKSPLVCAINNAFSRYSISDNDLFRFNKKMFARRRILLKKNRHKRAGHGAKNKLKPISILTGKSERFRKKLIERWACEIADFFIKNKVGTVQMENLESMKRKEDSYFNIRLRGFWPYAEMQNKIEFKLKQYGIEIRKVAPNNTSKTCSKCGHLNNYFNFEYRRKNKFPHFKCEKCNFKEDADYNAALNISNPKLKSTKEEP

SEQ ID NO: 1884 - protein, 726 aa, synthetic construct
SEVEFSHEYWMRRALTLAKRARDEREVPVGAVLVLNNRVIGVGWNRAVGLHDPTAHAEIMALRQGGLVMQNYRLVEATLYVTFEPCIMCAGAMIHSRIGRVVFGVRNSKRGAAGSLMNVLYYPGMNHRVEITEGILADECAALLCDFYRMPRQVFNARKKAQSSINPGGSSGGSSGSETPGTSESATPESSGGGSSGSAKNTITKTLQLRIVRPYNSAEVEKIVADEKNNREKIALEKNKDKVKEACSKHLKVASYCTTQVERNACPFCKARKLDDKFYQKLRGQFPDAVFWQELGEILRQLQKQAAEIYNQSLIELYYEIFIKGKGFANASSVEHYLSDVCYTRAAELFKNAAIASGLRGKVKSNFRLKELKNMKSGLPTTKSDNFPIPLVKQKGGQYTGFEISSHNDDFIIKIPFGRWQVKEEIDKYRPWEKFDFEQVRKIPKPISLLLSTQRRKRNKGWSKDEGTEAEIRKVMNGDYQTSYIEVKRGSKIGEKSAWMLNLSIDVPKIDKGVDPSIIGGIDVGVKSPLVCAINNALSRYSISDNDLFHFNKKMFARRRILLKKNRHKRAGHGAKNKLKPISILTEKSKRFRKKLIERWACEIADFFIKNKVGTVQMENLEGMKRKEDSYFNIRLRGFWPYAEMQNKIEFKLKQYGIEIRKVAPNNTSRTCSKCGHLNNYFNFEYRKMNKFPHFKCEKCNFKENADYNAALNISNPKLKSTKEEP

SEQ ID NO: 1885 - protein, 726 aa, synthetic construct
SEVEFSHEYWMRHALTLAKRARDEREVPVGAILVLNNRVIGEGWNRAIGLHDPTAHAEIMALRQGGLVMQNYRLTDATLYATFEPCVMCAGAMIHSRIGRVVFGVRNSKHGAAGSLMNVLNYPGMNHRVEITEGILADECAGLLCDFYRMPRQVFSARKKAQSSINPGGSSGGSSGGKAPGTSESATLESSGGSSGGSAKNSITKTLKLRIVRPYNSAEVEKIVADEKNNREKTALEKNKDKVKEACSKHLKVAAYCTTQVERNACLFCKARKLDDKFYQKLRGQFPDAVFWQEVGEIFRQLQKQAAEIYNQSLIELYYEIFIKGKGFANASSVEHYLSDVCYTRAAELFKNAAIASGLRGKVKSNFRLKELKNMKSGLPTTKSDNFPIPLVKQKGGQYTGFEISSHNDDFIIKIPFGRWQAKKEIDKYRPWEKFDFEQVRKSPKPISLLLSTQRRKRNKGWSKDEGTEAEIRKVMNGDYQTSYIEVKRGSKIGEKSAWMLNLSIDVPKIDKGVDPSIIGGIDVGVKSPLVCAINNAFNRYSISDNNLFHFNKKMFARRRILLKKNRHKRAGHGAKNKLRPISILTEKSERFRKKLIERWACEIADFFIRNKVGTVQMENLEGMKRKEDSYFNIRLRGFWPYAEMQNKIEFKLKQYGIEVRKVAPNNTSKTCSKCGHLNNYFNFEYRKKNKFPHFKCEKCNFKENADYNAALNISNPKLKSTKEEP

SEQ ID NO: 1886 - protein, 726 aa, synthetic construct
SEVEFSHEYWMRHALTLAKRARDEREVPVGAVLVLNNRVIGEGWNRAIGLHDPTAHAEIMALRQGGLVMQNHRLIDATLYVTFEPCVMCAGAMIHSRIGRVVFGVRNNKHGAAGSLMNVLNYPGMNHRVEITEGILVDECAALLCDFYRMPRQVFNARKKAQSSINPGGSFGGSSSSETPGTSESATLESSGGGSAGSTKNTITKTLKLRIVRPYNSAEVEKIMADEKNSREKIALEKNKDKVKEACSKHLKVAAYCTTQVERNACLFCKARKLDDRFYQKLRGQFPDAVFWQEIGEIFRQLQKQAAEVYNQSLVELYYEIFIKGKGVTNASRVEHYLSDVCYTRAAELFKNAAIASGLRSKVRSNFRLKELKNMKSGLPTTKSDNFPIPLVKQKGGQYTGFEISSHNDDFVIKIPFGRWQVKEEIDKYRPWEKFDFEQVRKSPKPISLLLSTRRRKRNKGWSKDEGTEAEIRRVMNGDYQTSYIEVKRGSKIGEKSAWMLSLSIDVPKIDKGVDPRIIGGIDVGVKSPLVCAISNAFSRYSISDNDLFHFNKKMFARRRILLKKSKHKRAGHGAKNKLKPITIMTEKSERFRKKLIERWACEIANFFIKNKVGTVQMENLEGMKRKEDSYFNIRLRGFWPYAEMQNKIEFKLKQYGIVVRKVAPNNTSKTCSKCGHLNNYFNFEFRKKNKFPHFKCEKCNFKENADYNAALNISNPKLKSTKEEP

SEQ ID NO: 1887 - protein, 726 aa, synthetic construct
SEVEFSHEYWMRHALTLAKRARDEREVPVGAILVLNNRVIGEGWNRAIGLHDPTAHAEIMALRQGGLVMQNHRLIDATLYVTFEPCVMCAGAMIHSRIGRVVFGVRNSKRGAAGSLMNVLDYPGMGHRVEITEGILADECAALLCDFYCMPRQVFNAQKRAQSSINSGGSSGGSSDSETPGTSESATPESSGGGSSGSAKDTITKTLQLRIVRPYNSAEVEKIVADEKNNREKIALEKNKDKVKEACSKHLKVASYCTTQVERNACPFCKARKLDDKFYQKLRGQFPDAMFWQELGEILRQLQKQAAEIYNQSLIELYYEIFIKGKGFANASSVEHYLSDVCYTRAAELFKNAAIASGLRGKVKSNFRLKELKNMKSGLPTTKSDNFPIPLVKQKGGQYAGFEISSHNDDFIIKIPFGRWQAKKEIDKYRPWEKFDFEQVRKSPKPISLLLSTQRRKRNKGWGKDEGTEAEIRKVMNGDYQTSYIEVKRGSKIGEKSAWMLNLSIDVPKIDKGVDPSIIGGIDVGVKSPLVCAINNALSRYSISDNDLFHFNKKMFARRRILLRKNRHKRAGHGARNKLKPITVLTEKSERFRKKLIERWACEIANFFIKNKVGTVQMENLESMKRREDSYFNIRLRGFWAYAEMQSKIEFKLKQYGIKIRKVAPNNTSKTCSKCGHLNNYFNFEFRKKNKFPHFKCEECNFKEDADYNAALNISNPKLKSTKEEP

SEQ ID NO: 1888 - protein, 726 aa, synthetic construct
SEAEFSHEYWMRHALTLAKRARDEREVPVGAVLVLNNRVIGEGWNRAIGLHDPTAHAEIMALRQGGLVIQNYRLTDATLYVTFEPCVMCAGAMIHSRIGRVVFGVRNSKRGAAGSLMNVLNYPGMNHCVEITEGILVDECAALLCDFYRMPRQVLNAQKKAQSSISSGGSSGGSSCSETPCASESVTPKSSGGGSSGSAKNTITKTLQLRIVRPYNSAEVEKIVADEKNNREKIALEKNKDKVKEACSKHLKVASYCTTQVERNACPFCKARKLDDKFYQKLRGQFPDAVFWQELGEILRQLQKQAAEIYNQSLIELYYEIFIKGKGLANTSSVEHYLSDVCYTRAAELFKNAAIASGLRGKVKSNFKLKELKSMKSGLPSTKSDNFPIPLVKQRGGQYTGFEISSHNDDFIIKIPFGRWQAKKEIDKYRPWEKFDFEQVRKSPKPISLLLSTQRRKRNRGWSKDEGTEAEIRKVMNGDYQTSYIEVKRGSKFGEKSAWMLNLSIDVPKIDKGVDPSIIGGIDVGVKSPLVCAINNAFSRYSISDNDLFRFNKKMFARRRILLGKNRHKRAGHGVKNKLKPITILTEKSGRFRKKLIERWACEIADFFVKNKVGTVQMENLESMKRKEDSYFNIRLRGFWPYAEMQNKIEFKLKQYGIKVRKVAPNNTSKTCSKCGHLNNYFNFEYRKKNKFPHFKCEKCNFKENADYNAALNISNPKLKSTKEEP

SEQ ID NO: 1889 - protein, 726 aa, synthetic construct
SEDEFSHEYWMRHALTLAKRARDGREVPVGAVLVLNNRVIGEGWNRAIGLHDPTAHAEIMALRQGGLVMQNYRLIDATLYVTFEPCVMCAGAMVHSRIGRVVFGVRNSKRGAAGSLMNVLDYPGMGHRVEITEGILADECAALLCDFYCMPRQVFNAQKRAQSSINSGGSSGGSSGSETPGTSESATPESSGGGSSGSTKNTITKTLQLRIVRPYNSAEVEKIVADEKNNREKIALEKNKDKVKEACSEHLKVAAYCTTQVERNACLFCKARKLDDRFYQKLRGQFPDAVFWQETGEIFRQLQRQAAEIYNQSLIELYYEIFIKGKGFANASSVEHYLSDVCYTRAAELFKNAAIASGLRGKVKSNFRLKELKNMKSGLPTTKSDNFPIPLVKQKGGQYTGFEISSHNDDFIIKIPFGRWQVKKEIDKYRPWEKFDFEQVRKSPKPISLLLSTQRRKRNKGWSKDEGTEAEIRKVMNGDYQTSYIEVKRGSKTGEKSAWMLNLSIDVPKIDKGVDPSIIGGIDVGVKSPLVCAINNAFSRYSISDNDLFRFNKKMFARRRILLKKNRHKRAGHGAKNKLKPISILTGKGERFRKKLIERWACEIADFFIKNKVGTVQMENLESMKRKEDSYFNIRLRGFWPYAEMQNKIEFKLKQYGIEIRKVAPNNTSKTCSKCGHLNNYFNFEYRKKNKFPHFKCEKCNFKENADYNAALNISNPKLKSTKEKP

SEQ ID NO: 1890 - protein, 726 aa, synthetic construct
SEVEFSHEYWMRHALTLAKRARDEREVPVGAILVLNNRVIGEGWNRAIGLHDPTAHAEIMALRQGGLAMQNYRLIDATLYVTFEPCVMCAGAMIHSRIGRVVFGVRNSKHGAAGSLVNVLNYPGMNHRVEITEGILADECAALLCDFYRMPRQVFNARKRAQSSINPGGSSGGSSGSETPGTSESATPESSGGSSGGSARNTITKTLKLRIVRPYNSAEVEKIVADEKNNREKIALEKNKDKVKEACSKHLKVAAYCTTQVERNACLFCKARRLDDKFYQKLRGQFPDAVFWQEIGEIFRQLQKQAAEIYNRSLIELYYEIFIKGRGFANASSVEHYLSDVCYTRAAELFKNAAIASGLRGKVKSNFRLKELKNMKSGLPTTKSDNFPIPLVKQKGGQYTGFEISSHNDDFIIKIPFGRWRVKKEIDKYRPWEKFDFEQVRKSPKPISLLLSTQRRKRNKGWSKDEGTEAEIRKVMNGDYRTSYIEVKRGGKTGEKSAWVLNLSIDVPKIDKGVDPSIIGGIDVGVKSPLVCAINNAFSRYSISDNDLFRFNKKMFARRRILLKKNRHKRAGHGAKNKLKPISILTEKSKRFRKKLIERWACEIADFFVKNKVGTVQMENLESMKRKEDSYFNIRLRGLWPYAEMQNKIEFKLKQYGIEIRKVAPNNTSKTCSKCGHLNNYFNFEYRRKNKFPHFKCEKCNFKENADYNAALNISDPKLKSTKEER

SEQ ID NO: 1891 - protein, 726 aa, synthetic construct
SEVEFSHEYWMRHALTLAKRARDEREVPVGAILVLNNRVIGEGWNRAIGLHDPTAHAEIMALRQGGLVMQNYRLIDATLYVTFEPCVMCAGALIHSRIGRVVFGVRNSKHGAAGSLVNVLNYPGMNHRVEITEGILADECAALLCDFYRMPRQVFNARKKAQSSINPGGSSGGSSGSETPGTSESPTPESPGGSSGGSAKNTITKALQLRIVRPYNSAEVEKIVADEKNNREKIALEKNKDKVKEACSKHLKVASYCTTQVERNACPFCKARKLDDKFYQKLRGQFPDAVFWQELGEIFRQLQKQAAEIYNQSLIELYYEIFIKGKGFANASSVEHYLSDVCYTRAAELFKNAAIASGLRGKVKSNFRLKELKNMKSGLPTTKSDNFPIPLVKQKGGQYTGFEISSHNDDFVIKIPFGRWQVKKEIDKYRPWEKFDFEQVRKGPKPISLLLSTQRRKRNKGWSKDEGTEAEIRKVMSGDYQTSYIEVKRGSKTGEKSAWMLNLSIDVPKIDKGVDPSIIGGIDVGVKSPLVCAINNALSRYSISDNDLFHFNKKVFARRRILLKKNRHRRAGHGAKNKLKPITILSEKSKRFRKKLIERWACEIADFFIKNKVGTVQMENLESMKRKEDSYFNIRLRGFWPYAEMQNKIEFKLKQYGIEIRKVAPNNTSKTCSKCGHLNNYFNFEYRNKNKFPHFKCEKCNFKENADYNAALNISNPKLKSTKEEP

SEQ ID NO: 1892 - protein, 726 aa, synthetic construct
SEVEFSHEYWMRHALTLAKRARDEREVPVGAILVLNNRVIGEGWNRAIGLNDPTAHAEIMALRQGGLVMQNYRLIDATLYVTFEPCVMCAGAMIHSRIGRVVFGVRNNKHGAAGSLVNVLNYPGMNHRVEITEGVLADECAALLCDFYRMPRQVFNARKKAQSSINPGGSSGGSGGSETPGTSESATPESSGGSSGSSAKNTITKTLKLRIVRPYNSAEVEKIVADEKDNREKVALEKNKGKVKEACSEHLKVAAYCTTQVERNACLFCKARKLDDGFYQKLRGQFPDAVFWQEIGEIFRQLQKQAAEIYNQSLIELYYEIFIKGKGLANASRVEHYLSDVCYTRAAELFKNAAIASGLRSKIKSNFRLKELRNMKSGLPTTKSDNFPIPLVKQKGGQCTGFEISNHNSDFIIKIPFGRWQVKKEVDKYRPWEKFDFEQVRKSPKPISLLLSTQRRRRNKGWSKDEGTEAEIRKVMNGDYQASYIEVKRGSKIGEKSAWMLNLSIDVPKIDKGVDPSIIGGIDVGVKSPLVCAINNAFSRYSISDNDLFRFNKKMFARRRILLKKNRHKRAGHGAKNKLKPISILTEKSKRFRKKLIERWACEIADFFIKNKVGTVQMENLESMKRKEDSYFNIRLRGFWPYAEMQNKIEFKLKQYGIEIRKVAPNNTSKTCSKCGHLNNYFNFEYRKKNKFPHFKCEKCNFKENADYNAALNISNPKLKSTKEEP

SEQ ID NO: 1893 - protein, 726 aa, synthetic construct
SEDEFSHEYWMRHALTLAKRARDGHEVPVGAVLVLNNRVIGEGWNRAIGLHDPTAHAEIMALRQGGRVMQNYRLIDATLYVTFEPCVMCAGAMIHSRVGRVVFGVRNNKHGAAGSLVNVLNYPGMNHRVEITEGILADECAALLCDFYRMPRQVFNARKKAQSSTNPGGSSGGSSGSETPGTSESATPESSGGSSGGSAKNSITKTLKLRIVRPYNSAEVEKIVADEKNNREKTALEKNKGKVREACSKHLKVASYCTTQVERSACPFCKARKLDDKFYQKLGGQFPDAVFWQELGEILRQLQKQAAEIYNQSLIELYYEIFIKGKGFANASSVEHYLSDVCYTRAAELFKNAAIASGLRGKVKSNFRLKELKNMKSGLPTTKSDNFPIPLVKQKGGQYTGFEISSHNDDFIIKIPFGRWQVRKEIDKYRPWEKFDFEQVRKSPKPISLLLSTQRRKRNKGWSKDEGTEAEIRKVMNGDYQTSYIEVKRGSKIGEKSAWMLSLSIDVPKIDKGVDPRIIGGIDVGVRSPLVCAINNAFSRYSISDNDLFRFNKKMFARRRILLKKNRHKRAGHGAKNKLKPITIMTEKSGRFRKKLIERWACEIADFFIKNKVGTVQMENLESMKRKEDSYFNIRLRGFWPYAEMQNKIEFKLKQYGIEIRKVAPNNTSKTCSKCGHLNNYFNFEYRKKNKFPHFKCEKCNFKENADYNAALNISNPKLKSTKEEP

SEQ ID NO: 1894 - protein, 726 aa, synthetic construct
SEVEFSHEYWMRHALTLAKRARDEREVPVGAVLVLNNRVIGEGWNRAIGLHDPTAHAEIMALRQGGLVLQNYRLVDATLYVTFEPCVLCAGAMVHSRIGRVVFGARNSKRGAAGSLMNILNYPGMNHRVEITEGILADECAALLCDFYRMPRQVFNAQKKAQSSINTGGSSGGSSGSETPSTSESATPESSGGSSGGSVKNTITKTLQLRIVRPYNSAEVEKIVTDEKNNREKIALEKNKDKVKEACSKHLKMASYCTTQVERNACLFCKARKLDDRFYQKLRGQFPDAVFWQELGGIFRQLQKQAAEIYNQSLIELYYEIFIKGKGITNASRVEHYLSDVCYTRAAELFKNAAIASGLRSKVRSNFRLKELKNMRSGLPTTKSDNFPIPLVKQKGGQYTGFEISSHNSDFIIKIPFGRWQVKEEIDKYRSWEKFDFEQVRKSPKPISLLLSTQRRKKNKGWSKDEGTEAEIRRVMNGDYQTSYIEVKRGSKIGEKSAWMLNLSIDVPKIDKGVDPSIIGGIDVGVKSPLVCAINNSSSRYSICDNDLFRFNKKMFARRRILLKKNRHKRAGHGAKNKLKPITILTKKSERFRKKLIERWVCEVADFFIKNKVGTVQMENLESMKRKEDSYFNIRLRGFWPYAEMQNRIELKLKQYGIEIRRVAPNNTSRTCSKCGHLNNYFDFEYRKKSKFPHFKCEKCNFREDADYNAALNISNPKLKSTKEEP

SEQ ID NO: 1895 - protein, 726 aa, synthetic construct
SEVEFSHEYWMRHALTLAKRARDEREVPVGAILVLNNRVIGEGWNRAIGLHDPTAHAEIMALRQGGLVMQNYRLIDATLYVTFEPCVMCAGAMIHSRIGRVVFGVRNSKHGAAGSLVNVLNYPGMNHRVEITEGILADECAALLCDFYRMPRQVFNARKKAQSSINPGGSSGGSSGSETPGTSESATPESSGGSSGSSAKNTITKTLKLRIVRPYNSAEVEKIVADEKNNREKIALEKNKDKVKEACSRHLKVAAYCTTQVERNACLFCKARRLDDKFYQKLRGQFPDAVFWQEIGEIFRQLQKQAAEIYNQSLIELYYEIFIKGKGFANASSVEHYLSDVCYTRAAELFKNAAIASGLRGKVKSNFRLKELKNMKSGLPTTKSDNFPIPLVKQKGGQYTGFEISSHNDDFIIKIPFGKWQVKKEIDKYRPWEKFDFEQVRKSPKPISLLLSTQRRKRNKGWSKDEGTEAEIRKVMNGDYQTSYIEVKRGSKTGEKSAWMLNLSIDVPKIDKGVDPSIIGGIDVGVKSPLVCAINNALSRYSISDNDLFRFNKKMFARRRILLKKNRHKRAGHGAKNKLKPISILTGKSERFRKKLIERWACEIADFFIKNKVGTVQMENLESMKRKEDSFFNIRLRGFWPYAEMQNRIEFKLKQYGIEIRKVAPNNTSKTCSKCGHLNNYFNFEYRKKNKFPHFKCEKCNFKESADYNAALNISNPKLKSTKEES

SEQ ID NO: 1896 - protein, 726 aa, synthetic construct
SEVEFSHEYWMRHALTLAKRARDEREVPVGAVLVLNNRVIGEGWNRAIGLHDPTAHAEIMALRQGGLVMQNYRLVDATLYVTFEPCVLCAGAMVHSRIGRVVFGVRNSKRGAAGSLMNVLDYPGMNHRVEITEGILADECAALLCDFYRMPRQVLNAQKKAQSSISPGGSSDGSSGSETPGTSESATPESSGGGSSGSAKNTITKTLQLRIVRPYNSAEVEKIVADEKNNREKIALEKNKDKVREACNKHLKVASYCTTQVERNACPFCKARKLDDKFYQKLRGQFPDAVFWQELGEILRQLQKQAAEIYNRSLIELYYEIFIKGRGFANASSVEHYLSDVCYTRAAELFKNAAIASGLRGKVKSNFRLKELKNMKSGLPTTKSDNFPIPLVKQKGGQYTGFEISSHNDDFIIKIPFGRWQVKKEIDKYRPWERFDFEQVRKSPKPISLLLSTQRRKRNKGWSKDEGTEAEIRKVMNGDYQTSYIEVKRGSKTGEKSAWMLNLSIDVPKIDKGVDPSIIGGIDVGVKSPLVCAINNAFSRYSISDNDLFHFNKKMFARRRILLKKNRHKRAGHGAKNKLKPISILTEKSERFRKKLIEKWACEIADFFIKNKVGTVQMENLESIKRKEDSYFNIRLRGFWPYAEMQSKIEFKLKQYGIEIRKVVPNNTSKTCSKCGHLNNYFNFEYRKKNKFPHFKCEKCNFKENADYNAALNISNPKLKGTKEGP

SEQ ID NO: 1897 - protein, 726 aa, synthetic construct
GEVEFSHEYWMRHALTLAKRARDEREVPVGAVLVLNNRVIGEGWNRAIGLHDPTAHAEIMALRQGGLVMQNYRLVDATLYVTFEPCVLCAGAMVHSRIGRVVFGVRNSKRGAAGSLMNVLNYPGMNHRVEITEGILADECAALLCDFYRMPRQVFSARKKAQSSINSGGSSGGNSGNKTPGTSESATPESSGGSSGGSAKNTITKTLKLRIVRPYNSAEVEKIVADEKNNREKIALEKNEDKVKEACSKHLKVAAYCTTQVERNACLFCRARKLDDKFYQKLRGQFPDAVFWQEISEIFRQLQKQAAEIYNQSLIELYYEIFIKGKGFANASSVEHYLSDVCYTRAAGLFKNAAIASGLRGKVKSNFRLKELKNMKSGLPTTKSDNFPIPLVKQKGGQYTGFEISSLNDDFIIKIPFGRWQVKKEIDKYRPWEKFDFEQVRKSPKPISLLLSTQRRKRNKGWSKDEGTEAEIRKVMNGDYQTSYIEVKRGSKIGEKSAWMLNLSIDVPKIDKGVDPSIIGGIDVGVKSPLVCAINNALSRYSISDNDLFHFNKKMFARRRILLRKNRHKRAGHGAKNKLKPITMMTEKSKRFRKKLIERWACEIADFFIKNKVGTVQMENLESMKRKEDSYFNIRLRGFWPYAEMQNKIEFKLKQYGIVVRKVAPNNTSKTCSKCGHLNNYFNFEYRKKNKFPHFKCEKCNFKENADYNAALNISNPKLKSTKEEP

SEQ ID NO: 1898 - protein, 726 aa, synthetic construct
SEVEFSHEYWMRHALALAKRARDEREVPVGAVLVLNNRVIGEGWNRAIGLHDPTAHAEIMALRQGGLVMQNYRLIDATLYVTFEPCVMCAGAMIHSRIGRVVFGVRNSKHGAAGSLVNVLNYPGMNHRVEITEGILADECAALLCDFYRMPRQVFGARRKAQSSINPGGSSGGSSGSETPGTSESPTPESPGGSSGGSAKNTITKTLKLRIVRPYNSAEVEKIVADEKNNREKIALEKNKNKVKEACSKHLKVAAYCTTQVERNACLFCKARKLDDKFYQKLRGQFPDAVFWQEVGEIFRQLQKQAAEIYNQSLIELYYEIFIKGKGFANASSVEHYLSDVCYTRAAELFKNAAIASGLRGKVKSNFRLKELKNMKSGLPTTKSDNFPIPLVKQKGGQYTGFEISNRNDDFIIKIPFGRWQAKKEIDKYRPWEKFDFEQVRKSPKPISLLLSTQRRKRNRGWSKDEGTEAEIRKVMNGDYQTSYIEVKRGSNIGGKSAWMLNLTIDVPKIDKGVDPSIIGGIDVGVKSPLVCAINNAFSRYSISDNDLFRFNKKMFARRRILLGKNRHKRAGHGVKNKLKPITILTEKSGRFRKKLIERWACEIADFFVKNKVGTVQMENLESMKRKEDSYFNIRLRGFWPYAEMQNKIEFKLKQYGIEIRKVAPNNTSKTCSKCGHLNNYFNFEYRKRNKFPRFKCEKCNFKENADYNAALNISNPKLKSPKEEP

SEQ ID NO: 1899 - protein, 726 aa, synthetic construct
SEDEFSHEYWMRHALTLAKRARDGREVPVGAVLVLNNRVIGEGWNRAIGLHDPTAHAEIMALRQGGLVMQNYRLIDATLYVTFEPCVMCAGAMVHSRIGRVVFGVRNSKRGAAGSLMNVLDYPGMNHRVEITEGVLADECAALLSDFYRMPRRVFNAQKKAQSSINSGGSSGGGSGSETPSTSESTTPESSGGSSGGPAKNTITKTLKLRIVRPYNSAEVEKIVADEKNNREKTALEKNKDKVKEACSKHLKVAAYCTTQVERNACLFCKARKLDDKFYQKLRGQFPDAVFWQEVGEIFRQLQKQAAEIYNQSLIELYYEIFIKGKGFANASSVEHYLSDVCYTRAAELFKNAAIASGLRGKVKSNFRLRELKNMKSGLPTTKSDNFPIPLVKQKGGQYTGFEISNHNSDFIIKIPFGRWQVKKEINKYRPWEKFDFEQVRKSPKPICLLLSTQRRKRNKGWSKDEGTEAEIRKVMNGDYQTSYIEVKRGSKIGEKSAWMLNLSIDVPKIDKGVDPSIIGGIDVGVKSPLVCAINNSSSRYSICDNDLFRFNKKMFARRRILLKKNGHKRAGHGAKNKLKPITIMTEKSKRFRKKLIERWACEIADFFIKNKVGTVQMENLESMKRKEDSYFNIRLRGFWPYAEMQNKIEFKLKQYGIVVRKVAPNNTSKTCSQCGHLNNYFNFEYRKKNKFPYFKCEKCNFKENADYNAALNISNPKLKSTKGEP

SEQ ID NO: 1900 - protein, 726 aa, synthetic construct
SEVEFSHEYWMRHALTLAKRARDEREVPVGAVLVLNNRVIGVGWNRAIGLHDPAAHAEIMALRQGGLVTQNYRLTDATLYVTFEPCVMCAGAIIHSRIGRVVFGVRNSKRGAAGSLMNVLNYPGMNHRVEITEGILVDECAALLCDFYRMPRQVFNAQKKAQSNINPGGSSGGSSDSETPGTSENATPGSSGGSSGGSAKNTITKTLKLRIVRPYNSAEVEKIVADEKNNREKIALEKNKDKVKEACGKHLKVAAYCTTQVERNACLFCKARRLDDKFYQKLRGQFPDAVFWQEIGEIFRQLQKQAAEIYNQSLIELYYEIFIKGKGFANASSVEHYLSDVCYTRAAELFKNAAIASGLRGKVKSNFRLKELKNMKSGLPTTKSDNFPVPLVKQKGGQYTGFEISNHNSDFIIKIPFGRWQVKEEINKYRPWEKFDFEQVRKSPKPISLLLSTQRRKRNKGWSKDEGTEAEIRKVMNGDYQTSYIEVKRGSKTGEKSAWMLNLSIDVPKIDKGVDPSIIGGIDVGVKSPLVCAINNAFSRYSISDNDLFRFNKKMFARRRILLKKNRHKRAGHGAKNKLKPISILTGKSERFRKKLIERWACEIADFFIKNKVGTVQMENLESMKRRGDSYFNIRLRGFWPYAEMQNKIEFKLKQYGIEIRKVAPNNTSKTCSKCGHLNNYFNFEYRKKNKFPHFKCEKCNFKENADYNAALNISNPKLKSTKEEP

SEQ ID NO: 1901 - protein, 726 aa, synthetic construct
SEVEFSHEYWMRHALTLAKRARDEREVPVGAVLVLNNRVIGEGWNRTTGLHDPTAHAEIMALRQGGLAMQNYRLIDATLYVTFEPCVMCAGAMIHSRIGRVVFGVRNSKHGAAGSLVNVLNYPGMNHRVETTEGILADECAALLCDFYRMPRQVFNARKKAQSSINPGGLSGGSSGSVTPGTSESATPGSSGGSSGGSAKNTITKTLKLRIVRPYNSAEVEKIVADEKNNREKIALEKNKDKVKEACSKHMKVAAYCTTQVERNACLFCKARRLDDKFYQKLRGQFPDAVFWQEIGDIFRQLQKQAAEIYNQSLIELYYEIFIKGKGIANASSVEHYLSDVCYTRAAELFKNAAIASGLRNKIKSNFRLKELKSMKSGLPTTKSDNFPIPLVKQKGGQYTGFEISSHDDDFIIKIPFGRWRVKKEFDKYRPWEKFDFEQVRKSPKPISLLLSTQRRKRNKGWSKDEGTEAEIRKVMNGDYQTSYIEVKRGSKIGEKSAWMLNLSINVPKIDKGVDPSIIGGIDVGVKSPLVCAIDNAFSRYSISDNDLFHFNKKVFARRRILLKKNRHKRAGHGAKNKLKPITILTEKSKRFRKKLIERWACEIADFFIKNKVGTVQMENLEGMKRREDSYFNIRLRGFWPYAEMLNKIEFKLKQYGIEVRKVAPNNTSRTCSKCGHLNNYFNFEYRKKNKFPHFKCEKCNFKENADYNAALNISNPKLKSTKEKP

SEQ ID NO: 1902 - protein, 726 aa, synthetic construct
SEDEFSHEYWMRHALTLAKRARDGREVPVGAVLVLNNRVIGEGWNRAIGLHDPTAHAEIMALRQGGLVMQNYRLIDATLYVTFEPCVMCAGAMVHSRIGRVVFGVRNSKRGAAGSLMNVLDYPGMGHRVEITEGILADECAGLLCDFYCMPRQVFNAQKRAQSSINSGGSSGGSSGSETPGTSESATPESSGGSSGGSAKNTITKTLTLRIVRPYNSAEVEKIVADEKNNREKIALEKNKDKVKEACSEHLKVAAYCTTQVERNACLFCKARKLDDKFYQKLRGQFPDAVFWQEIGEIFRQLQKQAAEIYNQSLIELYYEIFIKGKGIANASSVGHYLSDVCYTRAAELFKNAAIASGLRGKIKSNFRLKELKNMKSGLPTTKSDNFPIPLVKQKGGQYTGFEISNHNGDFIIKIPFGRWQVKKEINKYRPWEKFDFEQVRKSPKPISLLLSTQRRKRNKGWSKDEATEAEIKKVMNGDYQISYIEVKRGSKIGEKSAWTLNLSVDVPKIDKGVDPSIIGGIDVGVRSPLVCAINNAFSRYSISDNDLFRFNKKMFARRRILLEKNRHKRAGHGVKNKLKPITIMTEKSKRFRKKLIERWACEIADFFIKNKVGTVQMENLESMKRKEDSYFNIRLRGFWPYAEMQNKIEFKLKQYGIEIRKVAPNNTSKTCSKCGHLNNYFNFEYRKKNKFPHFKCEKCNFKENADYNAALNISNPKLKSTKEGP

SEQ ID NO: 1903 - protein, 726 aa, synthetic construct
SEVEFSHEYWMRHALTLAKRARDGREVPVGAVLVLNNRVIGEGWNRAIGLHDPTAHAEIMALRQGGLVMQNYRLIDATLYVTFEPCVMCAGAMVHSRIGRVVFGVRNSKRGAAGSLMNVLDYPGMGHRVEITEGILADECAALLCDFYCMPRRVFNAQKRAQSSINSGGSSGGSSGSETPGTSESATPESSGGGSSGSAKNTITKTLQLRIVRPYNSAEVEKIVTDEKNNREKIALEKNKDKVKEACSKHLKMASYCTTQVERNACLFCKARKLDDKFYQKLRGQFPDAVFWQELGGIFRQLQKQAAEIYNQSLIELYYEIFIKGKGITNASRVEHYLSDVCYTRAAELFKNAAIASGLRSKVRSNFRLKELKNMKSGLPTTKSDNFPIPLVKQKGGQYTGFEISSHNSDFIIKIPFGRWQVKEEIDKYRPWEKFDFEQVRKSPKPISLLLSTQRRKRNKGWSKDEGTEAEVRKVMNGDYRTSYIEVKRGSKIGEKSAWMLNLSIDVPKIDKGVDPSIIGGIDVGVKSPLVCAINNSSSRYSICDNDLFRFNKKMFARRRILLKKNRHKRAGHGAKNKLKPITILTKKSERFRKKLIERWVCEVADFFIKNKVGTVQMENLESMKRKEDSYFNIRLRGFWPYAEMQNRIELKLKQYGIEIRRVAPNNTSRTCSKCGHLNNYFNFEYRKKNKFPHFKCEKCNFKENADYNAALNISNPKLKSTKEEP

SEQ ID NO: 1904 - protein, 726 aa, synthetic construct
SEVEFSHEYWMRHALTLARRARDEREVPVGAILVLNNRVIGEGWNRAIGLHDPTAHAEIMALRQGGLVLQNYRLIDATLYVTFEPCVMCAGAMIHSRIGRVVFGVRNNKHGAAGSLVNVLNYPGMNHRVEITEGILADECAALLCDFYRMPRQVFNARKKTQSSINPGGSSGGSSGSETPGTSESATPESSGGSSGSSAKNTITKTLKLRIVRPYNSAEVEKIVADEKNNREKIALEKNRDKVKEACSEHLKVAAYCTTQVERSACLFCKARKLDDKFYQKLRGQFPDAVFWQEIGEVFRQLQKQAAEIYNQSLIELYYEIFIKGKGFANASSVEHYLSDVCYTRAAKLFKNAAIASGLRGKVKSNFRLKELKNMKSGLPTTKSDNFPIPLVKQKGGQYTGFEISNHDSDFIIKIPFGRWQVKKEIDKYRPWEKFDFEQVRKSPKPISLLLSTQRRKRNKGWSKDEGTEAEIKKVMNGDYQTSYIEVKRGSKIGEKSAWMLNLSIDVPKIDKGVDPSITGGIDVGVKSPLVCAINNALSRYSISDNDLFHFNKKMFARRRILLKKNRRRRAGHGAKNKLKPISILTEKSKRFRKKLIERWACEIADFFIKNKVGTVQMENLESMKRKEDSYFNIRLRGFWPYAEMQNKIEFKLKQYGIEIRKVAPNNTSKTCSKCGHLNNYFNFEYRKMNKFPHFKCEKCNFKENADYNAALNISNPKLKSTKEEP

SEQ ID NO: 1905 - protein, 726 aa, synthetic construct
SEVEFSHEYWMRHALTLAKRARDEREVPVGAVLVLNNRVIGEGWNRAIGLHDPTAHAEIMALRQGGQVMQNYRLTDATLYVTFEPCVMCAGAMIHGRIGRVVFGVRNSKRGAAGSLMNVLNYPGMNHCVEITEGILVDECAALLCDFYHMPRQVLNAQKKAQSSISSGGPSGGSSGSETPDTSESATPESSGGNSGGSAKDTITKTLKLRIVRPYNSAEVEKIVADEKNNREKIALEKNKDKVKEACSEHLKVAAYCTTQVERNACLFCKARKLDDKFYQKLRGQFPDAVFWQELGEIFRQLQKQTAEIYNQSLIELYYEILIKGKGFANASSVEHYLSDVCYTRAAELFKNAAIASGLRGKVKSNFRLKELKNMKSGLPTTKSDNFPIPLVKQKGGQYTGFEISSHSDDFIIKIPFGRWQVKEEIDKYRPWEKFDFEQVRKNPKPISLLLSTQRRKRNKGWSKDEGTEAEIRKVMNGDYQTSYIEVKRGSKIGEKSAWMLNLSIDVPKIDKGVDPSITGGIDVGVKSPLVCAINNAFSRYSISDNDLFRFNKKVFARRRILLKKNRHKRAGHGTKNKLKPITILTEKSGRFRKKLIERWACEIANFFIKNKVGTVQMENLESMKRKEDSYFNIRLRGFWPYAEMQNKIEFKLKQYGIKIRKVAPNNTSRTCSKCGHLNNYFSFEYRKKNKFPHFKCEKCNFKEDADYNAALNISNPKLKSTKEEP

SEQ ID NO: 1906 - protein, 726 aa, synthetic construct
SEVEFSHEYWMRHALTLAKRARDEREVPVGAVLVLNNRVIGEGWNRAIGLHDPTAHAEIMALRQGGLVMQNYRLIDATLYVTFEPCVMCAGAMTHSRIGRVVFGVRNSKHGAAGSLMNVLNYPGMNHRVEITEGILVDECAALLCDFYRMPRQVFNAQKKAQSSINSGGSSGGSSGSETPSTSESATPENSGGSSGGSAKNTITKTLQLRIVRPYNSAEVEKIVTDEKNNREKIALEKNKDKVKEACSKHLKMASYCTTQVERNACLFCKARKLDDKFYQKLRGQFPDAVFWQELGGIFRQLQKQAAEIYNQSLIELYYEIFIKGKGITNASRVEHYLSDVCYTRAAELFKNAAIASGLRSKVRSNFRLKELKNMKSGLPTTKSDNFPIPLVKQKGGQYTGFEISSHNSDFIIKIPFGRWQVKEEIDKYRPWEKFDFEQVRKSPKPISLLLSTQRRKKNKGWSKDEGTEAEIRRVMNGDYQTSYIEVKRGSKIGEKSAWMLNLSIDVPKIDKGVDPSIIGGIDVGVKSPLVCAINNSSSRYSICDNDLFRFNKKMFARRRILLKKNRHKRAGHGAKNKLKPITILTKKSERFRKKLIERWVCEVADFFIKNKVGTVQMENLESMKRKEDSYFNIRLRGFWPYAEMQNRIELKLKQYGIEIRRVAPNNTSRTCSKCGHLNNYFNFEYRKKSKFPHFKCEKCNFREDADYNAALNISNPKLKSTKEEP

SEQ ID NO: 1907 - protein, 726 aa, synthetic construct
SEVEFSHEYWMRHALTLAKRARDEREVPVGAVLVLNNRVIGEGWNRAIGLHDPTAHAEILALRQGGLVMQNYRLTDATLYVTFEPCVMCAGAMIHSRIGRVVFGVRNSKRGAAGSLMNVLDYPGMNHRVEITEGILADECAALLCDFYRMPRQVFNAQKKARSNINPGGSSGGSSGSETPGTSEGAIRESSGGSSGGSAKNTITKTLQLRIVRPYNSAEVEKIVADEKNSREKIALEKNKDKVKEACGKHLKVASYCTTQVERNACLFCKARKLDDKFYQKLRGQFPDAVFWQELGEIFRQLQKQAAEIYNQSLVELYYEIFIKGKGLANASSVEHYLSDVCYTRAAELFKNAAIASGLRGKVKSNFKLKELKSMKSGLPSTKSDNFPIPLVKQKGGQYTGFEISSRNDDLIIKIPFGRWQVKKEIDRYRPWEKFDFEQVRKSPKPISLLLSTQRRKRNKGWSKDEGTEAEIRKVMNGDYQTSYIEVKRGSKAGEKSAWMLSLSVDVPKIDKGVDPSIIGGIDVGVKSPLVCAINNALSRYSISDNDLFHFNKKMFARRRILLRNNRHKRAGHGAKSKLKPITILTEKGERFRKKLIERWACEIANFFVKNKVGTVQMENLESMKRKEDSYFNVRLRGFWPYAEMQNKIEFKLKQYGIGIRKVAPNNTSKTCSRCGHLNNYFNFEYRRKNKFPYFKCEKCNFKENADYNAALNISNPKLKNTKEEP

SEQ ID NO: 1908 - protein, 726 aa, synthetic construct
SEVEFSHEYWMRHALTLAKRARDEREVPVGAVLVLNNRVIGEGWNRAIGLHDPTAHAEIMALRQGGLVMQNYRLTDATLYVTFEPCVMCAGAMIHSRIGRVVFGVRNSKRGAAGSLMNVLNYPGMNHRVEITEGILVDECAALLCDFYRMPCQVLNAQKKAQSSISSGGSSGGSSGGDTLGASESVTPKSSVGSSASSTKNTITKTLKLRIVRPYNSAEVEKIVADEKDNREKIALEKNKDKVKEACSKHLKVAAYCTTQVERNACLFCKARKLDDKFYQKLRGQFPDAVFWQEIGEIFRQLQKQAAEIYNQSLIELYYEIFIKGKGFANASSVEHYLSDVCYTRAAGLFKNAAIASGLRGKVKSNFRLKELKNMKSGLPTTKSDNFPIPLVKQKGGQYTGFEISNHNSDFIIKIPFGRWQAKKEIDRYRPWEKFDFEQVRKSPKPISLLLSTQRRKRNKGWSKDEGTEAEIRKVMNGDYQTSYIEVKRGSKTGEKSAWMLNLSIDVPKIDKGVDPSIIGGIDVGVKSPLVCAINNAFSRYSISDNDLFRFNKKMFARRRILLKKNRHKRAGHGAKNKLKPISILTGKSGRFRKKLIERWACEIADFFIKNKVGTVQMEDLESMKRKEDSYFNIRLRGFWPYAEMQNKIEFKLKQYGIKIRRVAPNNTSKTCSKCGHLNNYFGFEYRKKNKFPPFKCEKCNFKEDADYNAALNISNPKLKSPKEEP

SEQ ID NO: 1909 - protein, 726 aa, synthetic construct
SEVEFSHEYWMRHALSLAKRARDEREVPVGAVLVLNNRIIGEGWNRAIGLHDPTAHAEIMALRQGGLVMQNYRLTDATLYVTFEPCVMCAGAMVHSRIGRVVFGVRNSKRGAAGSLMNVLNYPGVNHCVEITEGILVDECAALLCDFYRMPRQVLNAQKKAQSSISSGGSSGGCSGSEMPGASESVTPESSGGSSAGSTKNTITKTLKLRIVRPYNSAEVEKIVADEKNSREKIALERNKDKVKEACSEHLKVAAYCTTQVERNACLFCKARRLDDKFYQKLRGQFPDAVFWQEISEIFRQLQKQAAEIYNQSLIELYYEIFIKGKGFANASSVEHYLSDVCYARAAERFKNAAIASGLRGKVKSNFRLKELKNMKSGLPTTKSDNFPIPLVKQKGGQYTGFEISSHNDDFIIKIPFGRWQVKKEIDKYRPWEKFDFEQVRKSPKPISLLLSTQRRKRNKGWGKDEGTEAEIRKVMNGDYQTSYIEVKRGSKIGEKSAWMLNLSIDVPKIDKGVDPRIIGGIDVGVKSPLVCAINNAFSRYSISDNDLFHFNKKMFARRRILLRKNRHKRAGHGAKNKLKPITIMTEKSKRFRKKLIERWACEIADFFIKNKVGTVQMENLESMKRREDSYFNIRLRGFWPYAEMQNKIEFKLKQYGIVVRKVAPNNTSKTCSKCGHLNNYFNFEYRKKNKFPHFKCEKCNFKEDADYNAALNISNPKLKSTKGEP

SEQ ID NO: 1910 - protein, 726 aa, synthetic construct
SEVEFSHEYWMRHALTLAKRARDEREVPVGAILVLNNRVIGEGWNRAIGLHDPTAHAEIMALRQGGLVMQNYRLIDATLYVTFEPCVMCAGAMIHSRIGRVVFGVRNSKHGAAGSLVNVLNYPGMNHRVEITEGILADECAALLCDFYRMPRQVFNARKKAQSSINPSGSSGGSSGSVTPGTSESPTPESPGGSSGGSAKNTITKTLKLRIVRPYNSAEVEKIVADEKNNREKIALEKNKDKVKEACSKHLKVASYCTTQVERNACLFCRARKLDDKFYQKLRGQFPDAVFWQELGEIFRQLQKQAAEIYNQSLIELYYEIFIKGKGFANASSVEHYLSDVCYTRAAELFKNAAIASGLRGKVKSNFRLKELKNMKSGLPTTKSDNFPIPLVKQKGGQYTGFEISSHNDDFIIKIPFGRWQVKKEIDKYRPWEKFDFEQVRRSPKPISLLLSTQRRKRNKGWSKDEGTEAEIRKVMNGDYQTSYIEVKRGSKTGEKSAWMLNLSIDVPKIDKGVDPSIIGGIDVGVKSPLVCAINNAFSRYSISDNDLFRFNKKMFARRRILLKKNRHKRAGHGAKNKLKPISILTGKSERFRKKLIERWACEIADFFIKNKVGTVQMENLESMKRKEDSYFNIRLRGFWPYAEMQNRIELKLKQYGIEIRRVAPSNTSRTCSKCGHLNNYFNFEYRKKNKFPHFKCEKCNFREDADYNAALNISNPKLKSTKEEP

SEQ ID NO: 1911 - protein, 726 aa, synthetic construct
SEVEFSHEYWMRHALTLAKRARDEREVPVGAILVLNNRVIGEGWNRAIGLHDPTAHAEIMALRQGGLVMQNYRLIDATLYVTFEPCVMCAGAMIHSRVGRVVFGVRNSKHGAAGSLMNVLNYPGMNHRVEITEGILADECAALLCDFYRMPRRVFNARKKAQSSIDPGGPSGSSSSSETPGTSESATPESSGGSSGGSAKNTITKTLKLRIVRPYNSTEVEKIVADEKNNREKIALEKNKDKVKEACSKHLKVASYCTTQVERNACLFCKARKLDDKFYQKLRGQFPDAVFWQEIGEIFRQLQKQAAEIYNQSLIELYYEIFIKGKGFANASSVEHYLSDVCYTRAAELFKNAAIASGLRGKVRSNFRLKELKNMKSGLPTTKSDNFPIPLVKQKGGQYTGFEISNHNSDFIIKIPFGRWQAKKEIDKYRPWEKFDFEQVRKSPKPISLLLSTQRRKRNRGWSKDESTEAEIKKVMNGDYQTSYIEVKRGSKVGEKSAWMLNLSIDVPKIDKGVDPSIIGGIDVGVKSPLVCAINNALSRYSISDNDLFHFNKKMFARRRILLRKNRHKRAGHGAKNKLKPITIMTEKSKRFRKKLIERWACEIADFFIKNKVGTVQMENLESMKRREDSYFNIRLRGFWPYAEMQNKIEFKLKQYGIVVRKVAPNNTSKTCSKCGHLNNYFNFEYRKRNKFPHFKCEKCNFKENADYNAALNISNPKLKSTKEEP

SEQ ID NO: 1912 - protein, 726 aa, synthetic construct
SEVEFSHEYWMRHALALAKRARDEREVPVGAVLVLNNRVIGEGWNRAIGLHDPTAHAEIMALRQGGLVTQNYRLTEATLYVTFEPCVMCAGAMIHSRIGRVVFGVRNSKHGAAGSLVNVLNYPGMNHRVEITEGILADECAALLCDFYRMPRQVFNARKKAQSSINPGGSSGGSSGSETPGTSESAAPESSGGIPGGSAKNTITKTLKLRIVRPYNSAEVEKIVADEKNNREKIALERNKDKVKEACSKHLKVAAYCTTQVERNACLFCKARKLDDKFYQKLRGQFPDAVFWQEIGEIFRQLQKQAAEIYNQSLIELYYEIFIKGKGFANASSVEHYLSDVCYTRAAELFKNAAIASGLRGKVKGNFRLKELKNMKSGLPTTKSDNFPIPLVKQKGGQYTGFEISSHNDDFIIKIPFGRWQAKKEIDKYRPWEKFDFEQVRKSPKPISLLLSTQRRKRNEGWSKDEGTEAEIRKVMNGDYQTSYIEVKRGSKIGEKSAWMLNLSIDVPKIDKGVDPSIIGGIDVGVKSPLVCAINNAFSRYSISDNDLFRFNKKMFARRRILLGRNRHKRAGHGVKNKLKPITILTEKSGRFRKKLIERWACEIADFFVKNKVGTVQMENLESMKRKEDSYFNIRLRGFWPYAEMQNKIEFKLKQYGIKVRKVAPNNTSKTCSKCCHLNNYFSFEYRKKNKFPHFKCEKCNFKENADYNAALNISNPKLKSTKEEL

SEQ ID NO: 1913 - protein, 726 aa, synthetic construct
SEVEFSHEYWMRHALTLAKRARDEREVPVGAVLVLNNRVIGEGWNRTTGLHDPTAHAEIMALRQGGLVMRNYRLTDATLYVTFEPCVMCAGAMIHSRIGRVVFGVRNSKRGAAGSLMNVLNYPGMNHCVEITEGILVDECAALLCDFYRMPRQVLNAQKKAQSSISPGGSSGGSSGSKTPGASESVTPKSSGGSSGGSAKDTITKTLKLRIVRPYNSAEVEKIVADEKNNREKIALEKNKGKVKEACSKHLEVAAYCTTQVERNACLFCKARRLDDKFYQRLRGQFPDAVFWQEIGEIFRQLQKQTAEIYNQSLIELYYEIFIKGKGFANASSVEHYLSDVCYTRAAELFKNAAIASGLRGKVKSNFRLKELKNMKSGLPTTKSDNFPIPLVKQKGGQYTGFEISNHNSDFIIKIPFGRWQEKEEIDKYRPWEKFDFEQVRKSPKPISLLLSTQRRKRNKGWSKDEGTEAEIRRVMNGDYQTSYIEVKRGSKIGEKSAWMLNLSIDVPKIDKGVDPSIIGGIDVGVKSPLVCAINNSFSRYSICDNDLFHFNKKMFARRRILLKKNRHKRAGHGAKNKLKPITILTGKSERFRKKLIERWACEIADFFIKNEVGTVQMENLESMKRKEDSYFNIRLRGFWPYAEMQNKIEFKLKQYGIEVRKVAPNNTSKTCSKCGHLNNYFNFEYRKKNKFPHFKCEKCNFKENADYNAALNISNPKLKSTKEEP

SEQ ID NO: 1914 - protein, 726 aa, synthetic construct
SEVEFSHEYWMRHALTLAKRARDEREVPVGAVLVLNNRVIGEGWNRAIGLHDPTAHAEIMALRQGGLVLQNYRLVDATLYVTFEPCVLCAGAMVHSRIGRVVFGARNSKRGAAGSLMNILNYPGMNHRVEITEGILADECAALLCDFYRMPRQVFNAQKKAQSSINSGGSSSGSSGSETPSTSESATPESSGGSSGGSARNTITKTLQLRIVRPYNSAEVEKIVTDEKNNREKIALEKNKDKVKEACSKHLKMASYCTTQVERNACLFCKARKLDDKFYQKLRGQFPDAVFWQELGGIFRQLQRQAAEIYNQSLIELYYEIFIKGKGITNASRVEHYLSDVCYTRAAELFKNAAIASGLRSKVRSNFRLKELKNMKSGLPTTKSDNFPIPLVKQKGGQYTGFEISSHNSDFIIKIPFGRWQVKEEIDKYRPWEKFDFEQVRKSPKPISLLLSTQRRKRNKGWSKDEGTEAEIRKVMNGDYQTSYIEVKRGSKIGEKSAWMLNLSIDVPKIDKGVDPGIIGGIDVGVKSPLVCAINNASSRYSISDNDLFHFNKKMFARRRILLKKNRHKRAGHGAKNKLKPITIMTEKSKRFRKKLIERWACEIADFFIKNKVGTVQMENLESMKRKEDSYFNIRLRGFWPYAEMQNKIEFKLKQYGIEIRKVAPNNTSKTCSKCGHLNYYFNFEYRKRNKFPHFKCEKCNFKEDADYNAALNISNPKLKSTKEEP

SEQ ID NO: 1915 - protein, 726 aa, synthetic construct
SEVEFSHEYWMRHALTLAKRARDEREVPVGAILVLNNRVIGEGWNRAIGLHDPTAHAEIMALRQGGLVMQNYRLTDATLYATFEPCVMCAGAMIHSRIGRVVFGVRNSKHGAAGSLMNVLNYPGMNHRVEITEGILADECAGLLCDFYRMPRQVFSARKKAQSSINPGGTSGGSSGSETPGTNESPTPESSGGSPGGSAKNTITKTLKLRIVRPYNSAEVEKIVADEKNNREKIALEKNKDKVKEACSKHLKVAAYCTTQVERNACLFCKARKLDDKFYQKLRGQFPDAVFWQEIGEIFRQLQKQAAEIYNQSLIELYYEILIKGKGFANASSVEHYLSDVCYTRAAELFKNAAIASGLRNKVKSNFRLKELRNMKSGLPTTKSDNFPIPLVKQKGGQYTGFEISNHNGDFIIKIPFGRWQVKKVIDKYRPWEKFDFEQVRKSPKPISLLLSTQRRKRNKGWSKDEGTEAEIRKVMNGDYQTSYIEVKRGSKTGEKSAWMLNLSIDVPKIDKGVDPSIIGGIDVGVKSPLVCAINNAFSRYSISDNDLFRFNKKMFARRRILLKKNRHKRAGHGAKNKLKPISILTGKSERFRKKLIERWACEIADFFIKNKVGTVQMENLESMKRKEDSYFNIRLRGFWPYAEMQNRIEFKLKQYGIETRKVAPNNTSKTCSKCGHLNNYFNFEYRRKNKFPHFKCEKCNFKENADYNAALNISDPKLKSTKEEP

SEQ ID NO: 1916 - protein, 726 aa, synthetic construct
SEVEFSHEYWMRHALTLAKRARDEREVPVGAVLVLNNRVIGEGWNRAIGLHDPTAHAEVMALRQGGLVMQNYRLTDATLYVTFEPCVMCAGAMIHSRIGRVVFGVRNSKRGAAGSLMNVLNYPGMNHCVEITEGILVDECAALLCDFYRMPRQVLNAQKKAQPSISPGGSSGGSSGSETPGASGSVTPKSSGGSSAGSTKDTITKTLKLRIVRPYNSAEVEKTVADEKNSREKIALEKNKDKVKEACSEHLKVAAYCTTQVERNACLFCKARKLDDRFYQKLRGQFPDAVFWQEIGEIFRQLQKQAAEIYNQSLIELYYEIFIKGKGFANASSVEHYLSDVCYTRAAELFKNAAIASGLRGKVKSNFRLKELKNMRSGLPTTKSDNFPIPLVKQKGGQYTGFEISNHNSDFIIKIPFGRWQAKKEIDKYRPWEKFDFEQVRKSPKPISLLLSTQRRKKNRGWSKDEGTEAEIKKVMNGDYQTSYIEVKRGSKIGEKSAWMLNLSIDVPKIDKGVDPSIVGGIDVGVKSPLVCAISNAFSRYSISDNDLFHFNKKMFARRRILLKKSKHKRAGHGAKNKLKPITILTEKSRRFRKKLIERWACEIADFFIKNKVGTVQMENLESMKRREDSYFNIRLRGFWPYAEMQNKIEFKLKQYGIEIRKVAPNNTSKTCSKCGHLNNYFNFEYRKKNKFPHFKCEKCNFKENADYNAALNISNPKLKGTKEGP

SEQ ID NO: 1917 - protein, 726 aa, synthetic construct
SEVEFSHEYWMRHALTLAKRARDGREVPVGAVLVLNNRVIGEGWNRAIGLHDPTAHAEIMALRQGGLVMQNYRLIDATLYVTFEPCVMCAGAMVHSRIGRVVFGVRNSKRGAAGSLMNVLDYPGMNHRVEITEGILADECAALLCDFYCMPRQAFNAQKRAQSSINPGGSSGGSSGSETPGTSESATPESSGGGSSGSAKNTITKTLQLRIVRPYNSAEVEKIVADEKNNREKIALEKNKDKVKEACSKHLKVASYCTTQVERNACPFCKARKLDDKFYQKLRGQFPDAVFWQELGEILRQLQKQAAEIYNQSLIELYYEIFIKGRGFANACSVEHYLSDVCYTRAAELFKNAAIASGLRGKVKSNFRLKELKNMKSGLPTTKSDNFPIPLVKQKGGQYTGFEISSHNDDFIIKIPFGRWQVKKEIDKYRPWEKFDFEQVRKSPKPISLLLSTQRRKRNKGWSKDEGTEAEIRKVMNGDYQTSYIEVRRGSKIGEKNAWMLSLSIDVPKIDKGVDPSIIGGIDVGVKSPLVCAINNAFSRYSISDNDLFHFNKRMFARRRILLKKNRHKRAGHGAKNKLKPITILTEKSKRFRKKLIERWACEIADFFIKNKVGTVQMEDLESMKRRGDSYFNTRLRGLWPYAEMQNKIEFKLKQYGIEIRKVAPNNTSKTCSKCGHLNNYFNFEYRKKNKFPHFKCEKCNFKENADYNAALNISSPKLKNTKEEP

SEQ ID NO: 1918 - protein, 726 aa, synthetic construct
SEVEFSHEYWMRHALMLAKRARDEREVPVGAVLVLNNRVIGEGWNRAIGLHDPTAHAEIMALRQGGLVMQNYRLVDATLYVTFEPCVLCAGAMVHSRIGRVVFGVRNSKRGAAGSLMNVLNYPGMNHRVEITEGILADECAALLCDFYRMPHQVFNAQKRAQSSISPGGSSGGSSDSETPGASESVIPKSSGGSSGGSAKNTITKTLKLRIVRPYNSAEVEKIVADEKNNRERIALEKNKGKVKEACSKHLKVAAYCTTQVERNACLFCKARKLDDKFYQKLRGQFPDAVFWQEIGEIFRQLQRQAAEIYNQSLVELYYEIFIKGKGIANASSVEHYLSDVCYTRAAELFRNAAIASGLRNKIKSNFRLKELRNMKSGLPTTKSDNFPIPLVRQKGGQYTGFEISNHNGDFIIKIPFGGWQVKKEISKHRPWEKFDFEQVRKSPKPISLLLSTQRRKRNKGWGKDEGTEAEIRKVMNGDYQTSYIEVKRGSKIGEKSAWMLNLSIDVPKIDKGVDPSIIGGIDVGVKSPLVCAINNAFSRYSISDNDLFRFNKKMFARRRILLKKNRHKRAGHGAKNKLKPITVLTEKSVRFRKKLIERWACEIADFFIKNKVGTVQMENLESMKRKEDSYFNIRLRGFWPYAEMQNKIEFKLKQYGIEIRKVAPNNTSKTCSKCGHLNNYFSFEYRKKNKFPHFKCEKCNFKENADYNAALNISNPKLKSTKEEP

SEQ ID NO: 1919 - protein, 726 aa, synthetic construct
SEVEFSHEYWMRHALTLAKRARDEREVPVGAVLVLNNRAIGEGWNRAVGLHDPTAHAEIMALRQGGLVMQSYRLVDATLYVTFEPCVLCAGAMVHSRISRVVFGVRNSKRGAAGSLMNVLNNPGMNHRVEITEGILADECAALLCDFYRMPRQVFNAQKKARSNINSGSSSGGSSGSKTPGTSESATPEGSGGSSDGSAKNTITKTLKLRIVRPYNSAEVEKIVADEKNNREKIALEKNKDKVKEACSKHLKVASYCTTQVERNACLFCKARKLDDKFYQKLRGQFPDAVFWQELGEIFRQLQKQAAEIYNQSLIELYYEIFIKGKGFANASSVEHYLSDVCYTRAAELFKNAAIASGLRGKVKSNFRLKELKNMKSGLPTTKSDNFPIPLVKQKGGQYTGFEISSHNDDFVIKIPFGRWQVKKEIDKYRPWEKFDFEQVRKSPKPISLLLSTQRRKRNKGWSKDEGTEAEIRKVMNGDYQTSYIEVKRGSKIGEKSAWMLNLSIDVPKIDKGVDPSIIGGIDVGVKSPLVCAINNAFSRYSISDNDLFHFNKKMFARRRILLKKNRHKRAGHGAKNKLKPISILTEKSKRFRKKLIERWACEIADFFIKNKVGTVQMENLESMKRKEDGYFNIRLRGFWPYAEMQNKIEFKLKQYGIEIRKVAPNNTSKTCSKCGHLNNYFNFEYRKTNKFPHFKCEKCNFKEDADYNAALNISNPKLKSTKEEP

SEQ ID NO: 1920 - protein, 726 aa, synthetic construct
SEVEFSHEYWMRHALTLAKRARDEREVPVGAVLVLNNRVIGEGWNRAIGLHDPTAHAEIMALRQGGLALQNYRLVDATLYVTFEPCVLCAGAMVHSRIGRVVFGARNSKRGAAGSLMNILNYPGMNHRVEITEGILADECAALLCDFYRMPRQVFNAQEKAQSSINSGGSSGGSSGSETPSTSESATPESSGGSSGGSAKNTITKTLQLRIVRPYNSAEVEKIVTDEKNNREKIALEKNKDKVKEACSKHLKMASYCTTQVERNACLFCKARKLDDKFYQKLRGQFPDAVFWQELGGIFRQLQKQAAEIYNQSLIELYYEIFIKGKGITNASRVEHYLSDVCYTRAAELFKNAAIASGLRSKVRSNFRLKELKNMKSGLPTTKSDNFPIPLVKQKGGQYTGFEISSHNSDFIIKIPFGRWRVKEEIDKFRPWEKFDFEQVRKSPKPISLLLSTQRRKKNKGWSKDEGTEAEIRRVMNGDYQTSYIEVKRGSKIGEKSAWMLNLSIDVPKIDKGVDPSIIGGIDVGVKSPLVCAINNSSSRYSICDNDLFRFNKKMFARRRILLKKNRHKRAGHGAKNKLKPITILTKKSERFRKKLIERWVCEVADFFIKNKVGTVQMENLESMKRKEDSYFNIRLRGFWPYAEMQNRIELKLKQYGIEIRRVAPNNTSRTCSKCGHLNNYFNFEYRKKSKFPHFKCEKCNFREDADYNAALNISNPKLKSTKEEP

SEQ ID NO: 1921 - protein, 726 aa, synthetic construct
SEVEFSHEYWMRHALSLAKRARDEREVPVGAVLVLNNRIIGEGWNRAIGLHDPTAHAEIVALRQGGLVMQNNRLTGATLYVTFEPCVMCAGAMVHSRIGRVVFGVRNSKRGAAGSLMNVLNYPGVNHCVEITEGILVDECAALLCDFYRMPRQVLNAQKKAQSSISSGGSSGGCSGSEMPGASESVTPKSSGGSSAGSTKNTITKTLKLRIVRPYNSAEVEKIVADEKNSREKIALERNKDKVKEACSEHLKVAAYCTTQVERNACLFCKARKLDDRFYQKLRGQFPDAVFWQETGEIFRQLQRQAAEIYNQSLIELYYEIFIKGKGFANASSVEHYLSDVCYTRAAELFKNAAIASGLRGKVKSNFRLKELKNMKSGLPTTKSDNFPIPLVKQKGGQYTGFEISSHNDDFIIKIPFGRWQVKKEIDRYRPWEKFDFEQVRKSPKPISLLLSTQRRKRNKGWSKDEGTEAEIRKVMNGDYQTSYIEVKRGSKIGEKSAWMLSLSIDVPKIDKGVDPSTIGGIDVGVKSPLVCAINNAFCRYSISDNDLFHFNKKMFARRRILLKKSRHKRAGHGAKNKLKPISILTEKSKRFRKKLIERWACEIADFFIKNKVGTVQMENLESMKRKEDSYFNIRLRGFWPYAEMQNRIEFKLKQYGIEIRKVAPNNTSKTCSKCGHLNNYFNFEYRKKNKFPHFKCEKCNFKENADYNAALNISNPKLKSTKEEP

SEQ ID NO: 1922 - protein, 726 aa, synthetic construct
SEVEFSHEYWMRHALTLAKRARDEREVPVGAILVLNNRVIGEGWNRAIGQHDPTAHAEIMALRQGGLVMQNYRLIDATLYVTFEPCVMCAGAMIHSRIGRVVFGVRNSKHGAAGSLMNVLNYPGMNHRVEITEGILADECAALLCDFYHMPRQVFNGRKKAQSSINSGGSSGGSSGSETPGTSESATPESSGGSSSGSTKNTITKTLKLRIVRPYNSTEVEKIVADEKNNREKIALEKNKDKVKEACSRHLKVAAYCTTQVERNACLFCKARKLDDKFYQKLRGQFPDAVFWQEIGEIFRQLQKQAAEIYNQSLIELYYEIFIKGKGFANASSVEHYLSDVCYARAAELFKNAAIASGLRGKVKSNFRLKELKNMKSGLPTTKSDNFPIPLVKQKGGQYTGFEISSHNDDFIIKIPFGRWQVKEEIDKYRPWEKFDFEQVRKNPKPISLLLSTQRRKRNKGWSKDEGTEAEIRKVMNGDYQTSYIEVKRGSKIGEKSAWMLNLSIDVPKIDKGVDPSIIGGIDVGVKSPLVCAINNAFSRYSISDNDLFRFNKKVFARRRILLKKNRHKRAGHGTKNKLKPITMLTEKSGRFRKKLIERWACEIANFFIKNKVGTVQMENLESMKGKEDSYFNIRLRGFWPYAEMQNKIEFKLKQYGIKIRKVAPNNTSKTCSKCGHLNNYFSFEYRKMNKFPHFKCEKCNFKENADYNAALNISNPKLKSTKEEP

SEQ ID NO: 1923 - protein, 726 aa, synthetic construct
SEVEFSHEYWMRHALTLAKRARDEREVPVGAILVLNNRVIGEGWNRAIGLHDPTAHAEIMALRQGGLVMQNYRLIDATLYVTFEPCVMCAGAMIHSRIGRVVFGVRNNKHGAAGSLVNVLSYPGMNHRVEITEGILADECAALLCDFYRMPRRVFNAQKKAQSSINSGGSSGGGSGSETPSTSESTTPESSGGSSGGPAKNIITKTLKLRIVRPYNSAEVEKIVADEKNNREKIALEKNKDKVKEACSKHLRVASYCTTQVERNACPFCKARKLDDKFYQKLRGQFPDAVFWQELGEIFRQLQKQAAEIYNQSLIELYYEIFIEGKGSANARSVEHYLSDVCYTRAAELFKNAAIASGLRGKVKGNFRLKELKSMKSGLPTTKSDNFPIPLVKQKGGQYTGFEISSHNDDFIIKIPFGRWQVKKEIDKYRPWEKFDFEQVRKSPKPISLLLSTQRRKRNKGWSKDEGTEAEIRKVMNGDYQTSYIEVKRGRKIGERSAWMLNLSIDVPKIDKGVDPSIIGGIDVGVKSPLVCAINNALGRYSISDNDLFHFNKKVFARRRILLKKNRHKRAGHGTKNKLKPITILTEKSGRFRKKLIERWACEIANFFIKNKVGTVQMENLESMKRKEDSYFNIRLRGFWPYAEMQNKIEFKLKQYGIKIRKVAPNNTSKTCSKCGHLNNYFSFEYRKKNKFPHFKCEKCNFKEDADYNAALNISNPKLKSTKEEP

SEQ ID NO: 1924 - protein, 726 aa, synthetic construct
SEVEFSHEYWMRHALTLAKRARDEREVPVGAILVLNNRVIGEGWNRAIGLHDPTAHAEIMALRQGGLVMQNYRLVNATLYVTFEPCVMCAGAMIHSRIGRVVFGVRNSKRGAAGSLMNVLNYPGMNHRVEVTEGILTDECAALLCDFYRMPHQVLNAQKKAQSSINSGGSAGGSSGSETPGTSGSATPEGSGGSSGGSAKNTITKTLKLRIVRPYNSAEVEKIVADEKDNRERIALEKSKGKVKEACSKHLKVASYCTTQVERNACLFCKARKLDDKFYQKLRGQFPDAVFWQELGEIFRQLQKQAAEIYNQSLIELYYVIFIEGKGSANARSVEHYLSDVCYTRAAELFKNAAIASGLRGKVKGNFRLKELKSMKSGLPTTKSDNFPIPLVKQKGGQYAGFEISSHNDDFIIKIPFGRWQVKKEIDKYRPWEKFDFEQVRKSPKPISLLLSTQRRKRNKGWSKDEGTEAEIRKVMNGDYQTSYIEVKRGSKIGEKSAWMLNLSIDVPKIDKGVDPSIIGGIDVGVKSPLVCAINNAYSRYSISDNDLFHFNKKMFARRRILLKKTRHKRAGHGAKNKLKPVSILTEKSERFRKKLIERWACEIADFFIKNKVGTVQMENLESMKRREDSYFNIRLRGFWPYAKMQNKIEFKLKQYGIEIRKVAPNNTSKTCSKCGHLNNYFNFEYRKKNKFPHFKCEKCNFKENADYNAALNISNPKLKSTKEEP

SEQ ID NO: 1925 - protein, 726 aa, synthetic construct
SEVEFSHEYWMRHALTLAKRARDEREVPVGAVLVLNNRVIGEGWNRAIGLHDPTAHAEIMALRQGGLVMQNYRLSDATLYVTFEPCAMCAGAMIHSRIGRVVFGVRNSKRGAAGSLMNVLNFPGMNHCVEITEGILVDECAALLCDFYRMPRQVLSAQKKAQSSISSGGSSGGSSGSETPGASGSVTPKSSVGSSGGSAKNTITKTLKLRIVRPYNSAEVEKIVADEKNNREKIALEKNKDKVKEACSRHLKVAAYCTTQVERNACLFCKARKLDDRFYQKLRGQFPDAVFWQEISEIFRQLQKQAAEIYNQSLIELYYEIFIKGKGFANASSVEHYLSDVCYTRAAELFKNAAIASGLRGKVKSNFRLKELKNMKSGLPTTKSDNFPIPLVRQKGGQYTGFEISSHDDDFIIKIPFGRWQVKEEIVKYRPWEKFDFEQVRKSPKPISLLLSTQRRKRNKGWSKDEGTEAEIRKVMNGDYQTSYIEVKRGSKIGEKSAWMLNLSIDVPKIDKGVDPSIIGGIDVGVKSPLVCAINNAFSRYSISDNDLFRFNKKMFARRRILLKKNRHKRAGHGAKNKLKPISILTGKSERFRKKLIERWACEIADFFIKNKVGTVQMENLESMKRKEDSYFNIRLRGFWPYAEMQNKIEFKLKQYGIEIRKVAPNNTSKTCSKCGHLNNYFNFEYRKKNKFPHFKCEKCNFKENADYNAALNISNPKLKSTKEGP

SEQ ID NO: 1926 - protein, 726 aa, synthetic construct
SEVEFSHEYWMRHALTLAKRARDEREVPVGAVLVLNNRIIGEGWNRAIGLHDPTAHAEIMALHQGGLVMQNYRLIDATLYVTFEPCVMCAGAMIHSRIGRVVFGARNSKRGAAGSLMNVLSYPGMNHRVEITEGILADECAALLCDFYRMPRRVFNAQKKAQSSINSGGSSGGGSGSETPSTSESPTPESSGGSSGGPAKNTITKTLQLRIVRPYNSAEVEKIVADEKNNREKIALEKNKDKVKEACSKHLKVASYCTTQVERNACPFCKARKLDDKFYQKLRGQFPDAVFWQELGEILRQLQKQAAEIYNQSLIELYYEIFIKGRGFANAGSVEHYLSDVCYTRAAELFKNAAIASGLRGKVKSNFRLKELKNMKSGLPTTKSDNFPIPLVKQKGGQYTGFEISSHNDDFIIKIPFGKWQVKKEIDKYRPWEKFDFEQVRKSPKPISLLLSTQRRKRNKGWSRDEGTEAEIRKVMNGDYQTSYIEVKRGSKTGEKSAWMLNLSIDVPKIDKGVDPSIIGGIDVGVKSPLVCAINNAFSRYSISDNDLFRFNKKMFARRRILLKKNRHKRAGHGAKNKLKPISILTGKSERFRKKLIERWACEIADFFIKNKVGTVQMENLESMKRKEDSYFNIRLRGFWPYAEMQNKIEFKLKQYGIEIRKVAPNNTSKTCSKCGHQNNYFNFEYRKKNKFPHFKCEKCNYKEDADYNAALNISNPKLKSTKEEP

SEQ ID NO: 1927 - protein, 726 aa, synthetic construct
SEVEFSHEYWMRHALTLARRARDEHEVPVGAILVLNNRVIGEGWNRAIGLHDPTAHAEIMALRQGGLVMQNYRLVDATLYVTFEPCVMCAGAMIHSRIGRVVFGVRNNKHGAAGSLMNVLNYPGMNHRVEITEGILADECAALLCDFYRMPRQVFNARKKAQSSINPGGPSGGSSGSKTPGTSESASPKSSGGSPGSSAKNTITKTLRLRIVRPYNSAEVEKVVADEKNNREKIAMEKNKDKVREACSKHLKVASYCTTQVERNACLFCKARKLDDKFYQKLRGQFPDAVFWQELGGIFRQLQKQAAEIYNQSLIELYYEIFIKGKGITNASRVEHYLSDVCYTRAAELFKNAAIASGLRSKVRSNFRLKELKNMKSGLPTTKSDNFPIPLVKQKGGQYTGFEISSHNSDFIIKIPFGRWQEKEEIDKYRPWEKFDFEQVRKSPKPISLLLSTQRRKRNGGWSKDEGTEAEIRKVMNGVYQTSYIEVKRGSKTGEKSAWMLNLSINVPKIDKGVDPSIIGGIDVGVKSPLVCAINNALSRYSISDNDLFRFNKKMFARRRILLRKNRHKRAGHGAKNKLKPISILTGKSERFRKKLIERWACEIADFFIKNKVGTVQMENLESMKRKEDSYFNIRLRGFWPYAEMQNKIEFKLKQYGIEIRKVAPNNTSKTCSKCGHLNNYFSFEYRKKNKFPHFKCEKCNFKENADYNAALNICNPKLKSTKEEP

SEQ ID NO: 1928 - protein, 726 aa, synthetic construct
SEIEFSHEYWMRHALTLAKRARDEREVPVGAILVLNNRIIGEGWNRAIGLHDPTAHAEIMALRQGGLVMQNYRLSDATLYVTFEPCVMCAGAMIHSRIGRVVFGVRNSKRGAAGSLMNVLNYPGMNHCVEITEGILADECAALLCDFYRMPRQVFNARKKAQSSINPSGSSGGSSGSVTPGTSESATPESSSGGFGGSAKNTITKTLQLRIVRPYNSAEVEKIVADEKNNREKIALEKNKDKVEEACSKHLKVASYCTTQVERNACLFCKARRLDDKFYQKLRGQFPDAVFWQEIGEIFRQLQKQAAEIYNQSLVELYYEIFIKGKGIANASSVEHYLSDVCYTRAAELFKNAAIASGLRNKIKSNFRLKELRNMKSGLPTTKSDNFPIPLVKQKGGQYTGFEISSHNDDFVIKIPFGRWQVKEEIDKYRPWEKFDFEQVRKNPKPISLLLSTQRRKGNKGWSKDEGTEAEIRKVMNGDYQTSYIEVKRGSKIGEKGAWMLNLSIDVPKIDKGVDPSIIGGIDVGVKSPLVCAINNAFSRYSISDNDLFRFNKKVFARRRILLKKNRHKRAGHGTKNKLKPITILTEKSGRFRKKLIERWACEIANFFVKNKVGTVQMEDLESMKRKEDSYFNIRLRGFWPYAEMQNKIEFKLKQYGIKIRKVAPNNTSKTCSKCGHLNNYFNFEYRKKNKFPHFKCEKCNFKEDADYNAALNISNPKLKSTKEEP

SEQ ID NO: 1929 - protein, 726 aa, synthetic construct; identical to SEQ ID NO: 684

SEQ ID NO: 1930 - protein, 726 aa, synthetic construct
GEVEFSHEYWMRRALTLARRARDEREVPVGAILVLNNRVIGEGWNRAIGLHDPTAHAEIMALRQGGLVMQSYRLIDATLYVTFEPCVMCAGAMVHSRIGRVVFGVRNSKRGAAGSLMNVLDCPGMGHRVEITEGILADECAALLCDFYCMPRQVFNAQKRAQSSINSGGSSGGSSGSETPGTSESATPESSGGGSSGSAKNTITKTLQLRIVRPYNSAEVEKIVADEKNNREKIALEKNKDKVKEACSKHLKVAAYCTTQVERNACLFCKARRLDDKFYQKLRGQFPDAVFWQEIGEIFRQLQKQAAEVYNQSLVELYYEILIKGKGIANASSVEHYLSDVCYTRAAELFKNAAIASGLRNKIKSNFRLKELKNMKSGLPTTKSDNFPIPLVKQKGGQYTGFEISSHNSDFIIKIPFGRWQVKEEIDKYRPWEKFDFEQVRKSPKPISLLLSTQRRKKNKGWSKDEGTEAEIRRVMNGDYQTSYIEVKRGSKIGEKSAWMLNLSIDVPTIDKGVDPSIIGGIDVGVKSPLVCAINNSSSRYSICDNDLFRFNKKMFARRRILLKKNRHKRAGHGTKNKLKPITILTKKSERFRKKLIERWVCEVADFFIKNKVGTVQMENLESMKRKEDSYFNIRLRGFWPYAEMQNRIELKLKQYGIEIRRVAPNNTSRTCSKCGHLNNYFNFEYRKKNKFPHFKCEKCNFREDADYNAALNISNPKLKSTKEEP

SEQ ID NO: 1931 - protein, 726 aa, synthetic construct; identical to SEQ ID NO: 684

SEQ ID NO: 1932 - protein, 726 aa, synthetic construct
SEVEFSHEYWMRHALTLAKRARDEREVPVGAVLVLNNRVIGEGWNRAIGLHDPTAHAEIMALRQGGLVLQNYRLVDATLYVTFEPCVLCAGAMVHSRIGRVVFGARNSKRGAAGSLMNILNYPGMNHRVEITEGILADECAALLCDFYRMPRQVFNAQKKAQSSINSGGSSGGSSGSETPSTSESATPESSGGSSGGSAKNTITKTLQLRIVRPYNSAEVEKIVTDEKNNREKIALEKNKDKVKEACSKHLKVASYCTTQVERNACPFCKARKLDDKFYQKLRGQFPDAVFWQELGEILRQLQKQAAEIYNQSLIELYYEIFIKGRGFANASSVEHYLSDVCYTRAAELFKNAAIASGLRGKVKSNFRLKELKNMKSGLPTTKSDNFPIPLVKQKGGQYTGFEISSHNDDFIIKIPFGRWQVKKEIDKYRPWEKFDFEQVRKSPKPISLLLSTQRRKRNKGWSKDEGTEAEIRKVMNGDYQTSYIEVKRGSKTGEKSAWMLNLSIDVPKIDKGVDPCIIGGIDVGVKSPLVCAINNAFSRYSISDNDLFHFNKKMFARRRILLKENGHKRAGHGAKNKLKPITIMTEKSKRFRKKLIERWACEIADFFIKNKVGTVQMENLESMKRKEDSYFNIRLRGFWPYAEMQNKIEFKLKQYGIVVRKVAPNNTSKTCSKCGHLNNYFNFEYRKKNKFPHFKCEKCNFKENADYNAALNISNPKLKSTKGEP

SEQ ID NO: 1933 - protein, 726 aa, synthetic construct
SEVEFSHEYWMRHALTLAKRARDEREVPVGAVLVLNNRVIGEGWNRAIGLHDPTAHAEIMALRQGGLVMQNYRLIDATLYVTFEPCVMCAGAMIHSRIGRVVFGVRNNKHGAAGSLVNVLNYPGMNHRVEITEGILADECAALLCDFYRMPRQVFNARKKAQSSINPGGSSGGSSGSETPGTSESATPESSGGGFGGSAKNTITKTLQLRIVRPYNSAEVEKIVADEKNNREKIALEKNKDKVKEACSKHLKVASYCTTQVERNACLFCKARKLDDKFYQKLRGQFPDAVFWQELGEIFRQLQKQAAEIYNQSLIELYYEIFIKGKGIANASSVEHYLSDVCYTRAAELFKNAAIASGLRNKIKSNFRLKELRNMKSGLPTTKSDNFPIPLVRQKGGQYTGFEISNHNGDFIIKIPFGRWQVKKEISKHRPWEKFDFEQVRKSPKPISLLLSTQRRKKNKGWSKDEGTEAEIRRVMNGDYQTSYIEVKRGSKTGEKSAWMLSLSIDVPKVDKGVDPSIIGGIDVGVKSPLVCAINNAFSRYSISDNDLFRFNKKMFARRRILLKKSKHKRAGHGAKNKLKPITILTEKSGRFRKKLIERWACEIADFFIKNKVGTVQMENLEGMKRKEDSYFNIRLRGFWPYAEMQNKIEFKLKQYGIEIRKVAPNNTSKTCSKCGHLNNYFNFEYRKKNKFPHFKCEKCNFKENADYNAALNISNPMLKSTKEEP

SEQ ID NO: 1934 - protein, 726 aa, synthetic construct
SEVEFSHEYWMRHALTLAKRARDEREVPVGAILVLNNRVIGEGWNRAIGLHDPTAHAEIMALRQGGLVMQNYRLIDATLYVTFEPCVMCAGAMIHSRIGRVVFGARNSKHGAAGSLVNVLNYPGMNHRVEITEGILADECAALLCDFYRMPRQVFNAQKKAQPSISSGGSSGGSSGSETPGASESVTPKSSGGGSAGSTRNTITKTLKLRIVRPYNSAEVEKIVADEKNNREKIALEKNKDKVKEACSKHLKVAAYCTTQVERNACLFCKARKLDDKFYQKLRGQFPDAVFWQELGEIFRQLQKQAAEIYNQSLIELYYEILIKGKGFANACSVEHYLSDVCYTRAAELFKNAAIASGLRSKIKSNFRLKELKNMKSGLPTTKSDNFPIPLVKQKGGQYTGFEISNHNGDFIIKIPFGGWQVKKEIDKYRPWEKFDFEQVRKSPKPISLLLSTQRRKRNKGWSKDEGTEAEIRKVMNGDYQTSYIEVKRGSKTGEKSAWMVNLSIDVPKIDKGVDPSIIGGIDVGVKSPLVCAVNDALSRYSINDNDLFHFNKKMFARRRILLKKNGHKRAGHGTKNKLKPITTLTEKSKRFRKKLIERWACEIADFFIKNKVGTVQMENLESMKRKEDSYFNIRLRGFWPYAEMQNKIEFKLRQYGIEIRKVAPNNTSKTCSKCGHLNNYFDFEYRKKNKFPHFKCEKCYFKEDADYNAALNISNPRLKSTKEEP

SEQ ID NO: 1935 - protein, 726 aa, synthetic construct
SEVEFSHEYWMRHALTLAKRARDEREVPVGAVLVLNNRVIGVGWNRAIGLHDPTAHAEIMALRQGGLVMQNYRLTDATLYVTFEPCVMCAGAMVHSRIGRVVFGVRNSKRGAAGSLMNVLNYPGMSHCVEITEGILVDECAALLCDFYRMPRQVLNAQKKAQSSISSGGSSGGSGGGETPGASESVTPKSSGGSSAGSTKNTITKTLKLRIVRPYNSAEVEKIVADEKNSREKIALEKNKDKVKEACSEHLKVAAYCTTQVERSACLFCKARKLDDRFYQKLRGQFPDAVFWQEIGEIFRQLQKQAAEIYNQSLIELYYEIFIKGKGFANASSVEHYLSDVCYTRAAELFKNAAIASGLRGKVKSNFRLKELKNMKSGLPTTKSDNFPIPLVKQKGGQYTGFEISSHNDNFIIKIPFGRWQVKKEIDKYRPWEKFDFEQVRKSPKPISLLLSTQRRKRNKGWGKDEGTEAEIKKVMNGDYQTSYIEVKRGGKIGEKSAWMLNLSIDVPKIDKGVDPSIIGGIDVGVKSPLVCAINNAFSRYSISDNDLFRFNKKMFARRRILLKKSKHKRAGHGARNKLKPITILTEKSGRFRKKLIERWACEIADFFIKNQVGTVQMENLENMKRREDSYFNIRLRGFWPYAEMQNKIEFKLKQYGIEIRKVAPYNTSKTCSKCGHLNNYFNFEFRKKNKFPHFKCEKCNFKEDADYNAALNISNPKLKGTKEEP

SEQ ID NO: 1936 - protein, 726 aa, synthetic construct
SEVEFSHEYWMRHALTLAKRARDEREVPVGAILVLNNRVIGEGWNRAIGLHDPTAHAEIMALRQGGLVMQNYRLTDATLYVTFEPCVMCAGAMIHSRIGRVVFGVRNSKHGAAGSLVNVLNYPGMNHRVEITEGILADECAALLCDFYRMPRRVFNARMKAQSSISPGGSSGGSSGSDMPGTSESATPESSGGGSSGSARDTITKTLQLRIVRPYNSAEVEKIVADEKNNREKIALEKNKDKVREACSKHLKVASYCTTQVERNACPFCKARKLDDKFYQKLRGQFPDAVFWQELGEILRQLQKQAAEIYNQSLIELYYEIFIKGRGFANASSVEHYLSDVCYTRAAELFKNAAIASGLRGKVKGNFRLKELKNMKSGLPTTKSDNFPIPLVKQKGGQYTGFEISSHNDDFIIKIPFGRWQAKKEIDKYRPWEKFDFEQVRKSPKPISLLLSTQRRKRNRGWSEDEGTEAEIRKVMNGDYQTSYIEVKRGSKIGEKSAWMLNLSIDVPQIDKGVDPSIIGGIDVGVKSPLVCAINNAFSRYSISDNDLFRFNKKMFARRRILLGKNRHKRAGHGVKNKLKPITILTEKSGRFRKKLIERWACEIADFFVKNKVGTVQMENLESMKRKEDSYFNIRLRGFWPYAEMQNKIEFKLKQYGIKVRKVAPNNTSKTCSKCGHLNNYFSFEYRKKNKFPHFKCEKCNFKENADYNAALNISNPKLKSTKEEP

SEQ ID NO: 1937 - protein, 726 aa, synthetic construct
SEVEFSHEYWMRHALTLAKRARDEREVPVGAVLVLNNRVIGEGWNRATGLHDPTAHAEIMALRQGGLVMQNYRLFDATLYVTFEPCVMCAGAMIHSRIGRVVFGVRNSKRGAAGSLMNVLNYPGMDHRVEITEGILADECAALLCDFYRMPHQVFNAQKKAQSSINSGGSSDGSSGSVTPGPSESATPESSGGSSGGFAKSTITKTLKLRIVRPYNSAEVEKIVADEKNNREKIALEKNRDKVKEACSKHLKVAAYCTTQVERNACLFCKARKLDDRFYQKLRGQFPDAVFWQEVGEIFRQLQKQAAEIYNQSLIELYYEIFIKGKGFANASSVEHYLSDVCYTRAAELFKNAAIASGLRGKVKSNFRLKELKNMKSGLPTTKSDNFPIPLVKQKGGQYTGFEISNHNNDFIIKIPFGRWQVKKEINKYRPWEKFDFEQVRKGPKPISLLLSTQRRKRNKGWSKDEGTEAEIRKVMNGDYQTSYIEVKRGSRIGEKSAWMLSLSIDVPKIDRGVDPSIIGGIDVGVKSPLVCAINNALSRYSISDNDLFHFNKKMFARRRILLKKNRHRRAGHGARNKLKPITVLTGKSERFRKKLIERWACEIADFFIKNKVGTVQMENLESMKRKEDSYFNIRLRGFWPYAEMQNKIEFKLKQYGIEIRKVAPNNTSKTCSKCGHLNNYFNFEYRKKNKFPHFKCEKCSFKENADYNAALNISNPKLKNTKEEP

SEQ ID NO: 1938 - protein, 726 aa, synthetic construct
SEDEFSHEYWMRHALTLAKRARDEREVPVGAILVLNNRVIGEGWNRAIGLHDPTAHAEIMALRQGGLVMQNYRLIDATLYVTFEPCVMCAGAMIHSRIGRVVFGVRNNKHGAAGSLVNVLNYPGMNHRVGITEGILADECAALLCDFYRMPRQVFNARKKAQSSINPGGSSGGSSGSETPGTSESATPESSGGSSGGSAKNTITKTLKLRIVRPYNSAEVEKIVADEKNNREKIALEKNKDKVKEACSRHLKVAAYCTTQVERNACPFCKARKLDDKFYQKLRGQFPDAVFWQELGEILRQLQKQAAEIYNQSLIELYYEIFIKGRGFANASSVEHYLSDVCYTRAAELFKNAAIASGLRGKVKSNFRLKELKNMKSGLPTTKSDNFPIPLVKQKGGQYTGFEISSHNDDFIIKIPFGRWQVRKEIDKYRPWEKFDFEQVRKSPKPISLLLSTQRRKRNKGWSKDEGTEAEIRKVMNGDYQTSYIEVKRGSKTGEKSAWMLNLSIDVPKIDKGVDPSIIGGIDVGVKSPLVCAINNTFSRYSISDNDLFRFNKKMFARRRILLKKNRHKRAGHGAKNKLKPISVLTGKSERFRKKLIERWACEIADFFVKNKVGTVQMENLESMKRKEDSYFNIRLRGFWPYAEMQNKIEFKLRQYGIEIRKVAPNNTSKTCSKCGHLNNYFNFEYRKKNKFPHFKCEKCNFKENADYNAALNISNPKLKSTKEEP

SEQ ID NO: 1939 - protein, 726 aa, synthetic construct
SEVEFSHEYWMRRALTLAKRARDEREVPVGAILVLNNRVIGEGWNRAIGLHDPTAHAEIMALRQGGLVTQNYRLIDATLYVTFEPCVMCAGAMIHSRVGRVVFGVRNSKHGAAGSLMNVLNYPGMNHRVEITEGILADECAALLCDFYRMPRQVFNARKRAQSSINPGGSSGGSSGSETPGASESVTPKSSGGSSGGSAKNTITKTLKLRIVRPYNSAEVEKIVADEKNNREKIALEKNKGKVKEACSKHLEVAAYCTTQVERNACLFCKARKLDDKFYQKLRGQFPDAVFWQELGEIFRQLQRQAAEIYNQSLIELYYEIFIKGKGFANASSVEHYLSDVCYTRAAELFKNAAIASGLRGKVKSNFRLKELKNMKSGLPTTKSDNFPIPLVKQKGGQYTGFEISSHNDDFIIKIPFGRWQVRKEIDKYRPWEKFNFEQVRKSPKPISLLLSTQRRKRNKGWSKDEGTEAEIRKVMNGDYQTSYIEVKRGSKIGEKSAWMLNLSIDVPKIDKGVDPSIIGGIDVGVKSPLVCAINNAFNRYSISDNNLFHFNKKMFARRRILLKKNRHKRAGHGAKNKLKPISILTEKSERFRKKLIERWACEIADFFIRNKVGTVQMENLEGMKRREDSYFNIRLRGFWPYAEMQNKIEFKLKQYGIEVRKVAPNNTSKTCSKCGHLNNYFNFEYRKKNKFPHFKCEKCYFKEDADYNAALNISNPKLRSTKEEP

SEQ ID NO: 1940 - protein, 726 aa, synthetic construct
SEVEFSHEYWMRHALTLAKRARDEREVPVGAVLVLNNRVIGEGWNRAIGLHDPTAHAEIMALRQGGLVMQNYRLVDATLYVTFEPCVLCAGAMVHSRIGRVVFGVRNSKRGAAGSLMNVLDYPGMNHRVEVTEGILADECAALLCDYYRMPRQVFNARKKAQSSTNSGGSSDGGSGSETPGTSESATPESSGGSSGGSAKNTITKTLKLRIVRPYNSAEVEKIVADEKSNREKIALEKNKDKVKEACSEHLKVAAYCTTQVERSACPFCKARKLDDKFYQKLGGQFPDAVFWQEIGEIFRQLQKQAAEIYNQSLIELYYEIFIKGKGFANASSVEHYLSDVCYTRAAELFKNAAIASGLRGKVKSNFRLRELKNMKSGLPTTKSDNFPIPLVKQKGGQYTGFEISNHNSDFIIKIPFGRWQVKKEIDKFRPWEKFDFEQVRKSPKPISLLLSTQRRKRNKGWGKDEGTEAEIRKVMNGDYQTSYIEVKRGSKIGEKNAWMLNLSIDVPKIDKGVDPSIIGGIDVGVKSPLVCAINNAFSRYSISDNDLFHFNKKMFARRRILLKKSKHKRAGHGAKNKLKPITILTEKSGRFRKKLIERWACEIADFFIKNKVGTVQMEDLESMKRREDSYFNIRLRGFWPYAEMQSKIEFKLKQYGIKIRKVAPNNTSKTCSKCGHLNNYFSFEFRKKNKFPHFKCEKCNFKEDADYNAALNISNPKLKSTKEEP

SEQ ID NO: 1941 - protein, 726 aa, synthetic construct
SEVEFSHEYWMRHALTLAKRARDEREVPVGAILVLNNHVIGVGWNRAIGLHDPTAHAEIMALRQGGLVTQNYRLIDATLYVTFEPCVMCAGAMIHSRIGRVVFGVRNSKHGAAGSLVNVLNYPGMNHRVEITEGILADECAALLCDFYRMPRQVFNARKKAQSSINSGGSSGGSSGSETPGTSESATPKSSGGSSSGSAKNTITKTLQLRIVRPYNSAEVEKIVADEKNNREKIALEKNKDKVTEACSKHLKVAAYCTTQVERNACPFCKARRLDDKFYQKLRGQFPDAVFWQELGEIFRQLQKQAAEIYNQSLIELYYEIFIKGKGFANACSVEHYLSDVCYTRAAELFKNAAIASGLRGKVKSNFRLKELKNMKSGLPTTKSDNFPIPLVKQKGGQYTGFEISSHNDDFIIKIPFGRWQVKEEIDKYRPWEKFDFEQVRKNPKPISLLLSTQRRKRNKGWSKDEGTEAEIRKVMNGDYQTSYVEVKRGSKIGEKSAWMLNLSIDVPKIDKGVDPSIIGGIDVGVKSPLVCAINNAFSRYSISDNELFHFNKKMFARRRILLKKNRHKRAGHGARNKLKPITVLTEKSERFRKKLIERWACEIANFFIKNKVGTVQMENLESMRRREDSYFNIRLRGFWPYAEMQNKIEFKLKQYGIEIRKVAPNNTSKTCSKCGHLNNYFNFEFRKKNKFPHFKCEKCNFKENADYNAALNISNPKLKSTKEEP

SEQ ID NO: 1942 - protein, 726 aa, synthetic construct
SEVEFSHEYWMRHALTLAKRARDEREVPVGAVLVLNNRVIGEGWNRAIGLHDPTAHAEIMALRQGGLVMQNYRLSDATLYVTFEPCVMCAGAMIHSRIGRVVFGVRNSKRGAAGSLMNVLNYPGMNHCVEITEGILVDECAALLCDFYRMPRQVLSAQKKAQSSVSSGGSSGGSSGSETPGASGSVTPKSSVGSSAGSTKNTITKTLKLRIVRPYNSAEVERIVADEKNNREKIALEKNRDKVKEACSKHLKVAVYCTTQVERNACLFCKARKLDDKFYQKLRGQFPDAVFWQEINEIFRQLQKQAAEIYNQSLIELYYEIFIKGKGFANASSVEHYLSDVCYTRAAELFKNAAIASGLRGKVKGNFKLKELKNMKSGLPTTKSDNFPIPLVKQKGGQYTGFEISSHNDDFIIKIPFGRWQVKKEIDRYRPWEKFDFEQVRKSPKPISLLLSTQRRRRNKGWSKDEGTEAEIRKVMNGDYQTSYIEVKRGSKTGEKSAWMLNLSIDVPKIDKGVDPSIIGGVDVGVKSPLVCAINNAFSRYSISDNDLFRFNKKMFARRRILLKKNRHKRAGHGAKNKLKPISILTGKSERFRKKLIERWACEIADFFIKNKVGTVQMENLESLKRKEDSYFNIRLRGFWPYAEMQNKIEFKLKQYGIEIRRVAPNNTSRTCSKCGHLNNYFDFEYRRKYKFPHFKCEKCNFKENADYNAALNISNPKLKSTKEEP

SEQ ID NO: 1943 - protein, 726 aa, synthetic construct
SEVEFSHEYWMRHALTLAKRARDEREVPVGAVLVLNNRVIGEGWNRTTGLHDPTAHAEIMALRQGGLVMRNYRLTDATLYVTFEPCVMCAGAMIHSRIGRVVFGVRNSKRGAAGSLMNVLNCPGMNHCVEITEGILVDECAALLCDFYRMPRQVLNAQKKAQSSISPGGSSGGSSGSETPGASESVTPKSSGGSSGGSAKNTITKTLKLRIVRPYNSTEVEKIVADEKNNREKVALEKNKDKVKEACSKHLKVAAYCTTQVERNACLFCKARKLDDRFYQKLRGQFPDAVFWQEIGEIFRQLQKQAAEIYNQSLIELYYEIFIKGKGFANASSVEHYLSDVCYTRAAELFKNAAIASGLRGKVKSNFRLKELKNMKSGLPTTKSDNFPIPLVKQKGGQYTGFEISSHNDDFIIKIPFGRWQVKKEIDKYRPWEKFDFEQVRKSPKPISLLLSTQRRKRNKGWSKDEGTEAEIRKVMNGDYQTSYIEVKRGSKIGEKSAWMLNLSIDVPKIDKGVDPSIIGGIDVGVKSPLVCAINNAFSRYSISDNDLFHFNKKMFARRRILLKKSRHKRAGHGAKNKLKPISILTEKSKRFRKKLIERWACEIADFFIKNKVGTVQMENLESMKRKEDSYFNIRLRGFWPYAEMQNKIEFKLKQYGIVVRKVAPNNTSKTCSQCGHLNNYFNFEYRKKNKFPYFKCEKCNFKENADYNAALNISNPQLKSTKGEP

SEQ ID NO: 1944 - protein, 726 aa, synthetic construct
SEVEFSHEYWMRHALTLAKRARDEREVPVGAILVLNNRVIGEGWNRAIGLHDPTAHAEIMALRQGGLVMQNYRLIDATLYVTFEPCVMCAGAMIHSRIGRVVFGVRNNKHGAAGSLVNVLNYPGMNHCVEITEGILVDECAALLCDFYRMPRQVLSAQKKAQSSISPGGSSGGSSGSETPGASGSVTPKSSGGSSAGSTKDTITKTLKLRIVRPYNSAEVEKIVADEKNSREKIALEKNKDKVKEACSKHLKVASYCTTQVERNACLFCKARKLDDKFYQKLRGQFPDAVFWQELGGIFRQLQKQAAEIYNQSLIELYYEIFIKGKGITNASRVEHYLSDVCYTRAAELFKNAAIASGLRSKVRSNFRLKELKNMKSGLPTTKSDNFPIPLVKQKGGQYTGFEISNHNSDFIIKIPFGRWRVKEEIDKYRPWEKFDFEQVRKSPKPISLLLSTQRRKKNKGWSKDEGTEAEIRRVMNGDYQTSYIEVKRGSKIGEKSAWMLNLSIDVPKIDKGVDPSIIGGIDVGVKSPLVCAINNAFSRYSISDNDLFHFNKKMFAMRRILLKKNRHKRAGHGAKNKLKPITILTEKSKRFRKKLIERWACEIADFFIKNKVGTVQIENLESMKRKEDSYFNIRLRGFWPYAEMQNKIEFKLKQYGIEIRKVAPNNTSKTCSKCGHLNSYFNFEYRKKNKFPHFKCEKCNFKENADYNAALNISNPKLKSTKEEP

SEQ ID NO: 1945 - protein, 726 aa, synthetic construct
SEVEFSHEYWMRHALTLAKRARDEREVPVGAILVLNNRVIGEGWNRTTGLHDPTAHAEIMALRQGGLVMQNHRLVDATLYVTFEPCVMCAGAMIHSRIGRVVFGVRNSKRGAAGSLMNVLNYPGMNHCVEITEGILVDECAALLCDFYRMPRQVFNAQKKAQSSINSGGSSGGSSGSETPSTSESATPESSGGSSGGSAKNTITKTLQLRIVRPYNSAEVEKIVTDEKNNREKIALEKNKDKVKEACSKHLKMASYCTTQVERNACLFCKARKLDDKFYQKLRGQFPDAVFWQELGEILRQLQKQAAEIYNQSLIELYYEIFIKGRGFANASSVEHYLSDVCYTRAAELFKNAAIASGLRGKVKSNFRLKELKNMKSGLPTTKSDNFPIPLVKQKGGQYTGFEISSHNDDFIIKIPFGRWQVKKEIDKYRPWEKFDFEQVRKSPKPISLLLSTQRRKRNKGWSKDEGTEAEIRKVMNGDYQTSYIEVKRGSKIGEKSAWMLNLSIDVPKIDKGVDPSITGGIDVGVKSPLVCAINNAFSRYSISDNDLFRFNKKVFARRRILLRKNRHKRAGHGTKNKLKPITILTEKSGRFRKKLIERWACEIANFFIKNKVGTVQMENLESMKRKEDSYFNIRLRGFWPYAEMQNKIEFKLKQYGIKIRKVAPNNTSKTCSKCGHLNNYFSFEYRKKNKFPHFKCEKCNFKEDADYNAALNISNPKLKSTKEEP

SEQ ID NO: 1946 - protein, 726 aa, synthetic construct
SEVEFSHEYWMRHALTLAKRARDEREVPVGAILVLNNRVIGEGWNRAIGLHDPTAHAEIMALRQGGLVMQNYRLIDATLYVTFEPCVMCAGAMIHSRIGRVVFGVRNSKHGAAGSLVNVLNYPGMNHRVEITEGILADECAALLCDFYRMPRQVFGARRKAQSNINPGGSSGGSSSSETPGTSESPTPESPGGSSGGSAKNTITKTLKLRIVRPYNSAEVEKIVADEKNNREKIALEKNKGKVKEACSKHLEVAAYCTTQVERNACLFCKARKLDDKFYQKLRGQFPDAVFWQELGGIFRQLQKQAAEIYNQSLIELYYEIFIKGKGITNASRVEHYLSDVCYTRAAELFKNAAIASGLRSKVRSNFRLKELKNMKGGLPTTKSDNFPIPLVKQKGGQYTGFEISSHNDDLIIKIPFGRWQVKKEIDKYRPWEKFDFEQVRKSPKPISLLLSTQRRKRNKGWSKDEGTEAEIRKVMNGDYQTSYIEVKRGSKTGEKSAWMLNLSIDVPKIDKGVDPSIIGGIDVGVKSPLVCAINSAFSRYSISDNDLFRFNKKMFARRRILLKKNRHKRAGHGARNKLRPITVLTEKSERFRKKLIERWACEIANFFIKNKVGTVQMENLESMKRREDSYFNIRLRGFWPYAEMQSKIEFKLKQYGIKIRKVAPNNTSKTCSKCGHLNNYFNFEFRKKNKFPHFKCEKCNFKEDADYNAALNISNPKLKSTMEEP

SEQ ID NO: 1947 - protein, 726 aa, synthetic construct
SEVEFSHEYWMRHALTLAKRARDEREVPVGAILVLNNRVIGEGWNRAIGLHDPTAHAEIMALRQGGLVMQNYRLIDATLYVTFEPCVMCAGAMIHSRIGRVVFGVRNNKHGAAGSLVNVLDYPGMGHRVEITEGILADECAALLCDFYCMPRQVFNAQKKAESSINSSGSSGGSSGSETPGTSESATPESSGGGSSGSAKNTITKTLQLRIVRPYNSAEVEKIVADEKNNREKIALEKNKDKVKEACSRHLKVASYCTTQVERNACLFCKARKLDDKFYQKLRGQFPDAVFWQELGGIFRQLQKQAAEIYNQSLIELYYEIFIKGKGITNAGSVEHYLSDVCYTRAAELFKNAAIASGLRGKVKSNFRLKELKNMKSGLPTTKSDNFPIPLVKQKGGQYTGFEISNHNSDFIIKIPFGRWQVKKEINKYRPWEKFDFEQVRKSPKPISLLLSTQRRKRNKGWSKDEGTEAEIRKVMNGDYQTSYIEVKRGSKIGEKSAWMLNLSIDVPEIDKGVDPSIIGGIDVGVRSPLVCAINNAFSRYSISDNDLFRFNKKMFARRRILLKKNRHKRAGHGAKNKLKPISILTERSERFRKKLIERWACEIADFFIKNKVGTVQMENLESMKRKEDSYFNIRLRGFWPYAEMQNKIEFKLKQYGIEIRKVAPNNTSKTCSKCGHLNNYFNFEYRKKNKFPHFKCEKCNFKENADYNAALNISNPKLKSTKGEP

SEQ ID NO: 1948 - protein, 726 aa, synthetic construct
SEVEFSHEYWMRHALTLAKRARDEREVPVGAVLVLNNRVIGEGWNRTTGLHDPTAHAEIMALRQGGLVMQNHRLVDATLYVTFEPCVMCAGAMIHSRIGRVVFGVRNSKRGAAGSLTNVLNYPGMNHRVEITEGILVDECAALLCDFYRMPRQVFSAQKKAQSTINSGGSSGGSSGSETPGTSESPTPESSGGSPGGSAKNTITKTLKLRIVRPYNSAEVEKIVADEKNNREKIALEKNKDKVKEACSKHLKVASYCTTQVERNACPFCKARKLDDKFYQKLRGQFPDAVFWQELGEILRQLQKQAAEIYNQSLIELYYEIFIKGRGFANASSVEHYLSDVCYTRAAELFKNAAIASGLRGKVKSNFRLKELKNMKSGLPTTKSDNFPIPLVKQKGGQYTGFEISSHNDDFIIKIPFGRWQVKKEIDKYRPWEKFDFEQVRKSPKPISLLLSTQRRKGNKGWSKDEGTEAEIRKVMNGDYQTSYIEVKRGSKIGEKSAWMLNLSIDVPKIDKGVDPGIIGGIDVGVKSPLVCAINNAFSRYSISDNDLFRFNKKMFARRRILLKKNRHKRAGHGAKNKLKPISILTEKSERFRKKLIEKWACEIADFFIKNKVGTVQMENLESMKRREDSYFNIRLRGFWPYAEMQNKIEFKLKQYGIEIRKVAPNNTSKTCSKCGHLNNYFNFEYRKKNKFPHFKCEKCNFKENADYNAALNISNPKLKSTKEEP

SEQ ID NO: 1949 - protein, 726 aa, synthetic construct
SEDEFSHEYWMRHALTLAKRARDGREVPVGAVLVLNNRVIGEGWNRAIGLHDPTAHAEIMALRQGGLVMQNYRLIGATLYVTFEPCVMCAGAMVHSRIGRVVFGVRNSKRGAAGSLMNVLNYPGMNHRVEITEGILADECAALLCDYYRMPRQVFNARKKAQSSINSGGSSDGGSSSETPGTSESATPESSGGSSGGTAKNTITKTLKLRIVRPYNCAEVEKIVTDEKNNREKIALEKNKDKVKEACSKHLKMASYCTTQVERNACLFCKARKLDDKFYQKLRGQFPDAVFWQELGGIFRQLQKQAAEIYNQSLIELYYEIFIKGKGITNASRVEHYLSDVCYTRAAELFKNAAIASGLRSKVRSNFRLKELKNMKSGLPTTKSDNFPIPLVKQKGGQYTGFEISSHNSDFIIKIPFGRWQVKEEIDKYRPWEKFDFEQVRKSPKPISLLLSTQRRKKNKGWSKDESTEAEIRRVMNGDYQTSYIEVKRGSKIGEKSAWMLNLSIDVPKIDKGVDPSIIGGIDVGVKSPLVCAINNSSSRYSICDNDLFRFNKKMFARRRILLRKNRHKRAGHGARNKLKPITVLTEKSERFRKKLIERWACEIANFFIKNKVGTVQMENLESMKRREDSYFNIRLRGFWPYAEMQNKIEFKLKQYGIEIRKVAPSNTSKTCSKCGHLNNYFSFEYRKKNKFPHFKCKKCNFKENADYNAALNISNPKLKSTKEEP

SEQ ID NO: 1950 - protein, 726 aa, synthetic construct
SEVEFSHEYWMRHALTLAKRARDEREVPVGAVLVLNNRVIGEGWNRAIGLHDPTAHAEIMALRQGGLVIQNYRLSDATLYVTFEPCVMCAGAMIHSRIGRVVFGVHNSKRGAAGSLMNVLNYPGMNHCVEITEGILVDECAALLCDFYRMPRQVLSAQKKAQSSVSSGGSSGGSSGSETPGASGSVTPKSSVGSPAGSAKNTITKTLQLRIVRPYNSAEVEKIVADEKNNREKIALEKNKDKVKEACSKHLKVASYCTTQVERNACLFCKARKLDDKFYQKLRGQFPDAVFWQELGEIFRQLQKQAAEIYNQSLVELYYEIFIKGKGIANASSVEHYLSDVCYTRAAELFKNAAIASGLRNKIKSNFRLKELRNMKSGLPTTKSDNFPIPLVRQKGGQYTGFEISNHNGDFIIKIPFGRWQVKKEISKHRPWEKFDFEQVRKSPKPISLLLSTQRRKRNKGWGKDEGTEAEIRKVMNGDYQTSYIEVKRGSKIGEKSAWMLNLSIDVPKVDKGVDPNIIGGIDVGVKSPLVCAINNALSRYSISDNDLFHFNKKMFARRRILLRKNRYKRAGHGARNKLKPITVLTEKSERFRKKLIERWACEIANFFIKSKVGTVQMEDLESMKRREDSYFNIRLRGFWPYAEMQNKIEFKLKQYGIEIRKVAPNNTSKTCSKCGHLNNYFNFEYRKMNKFPHFKCEKCNFKENADYNAALNISNPKLKSTKEEP

SEQ ID NO: 1951 - protein, 726 aa, synthetic construct
SEVEFSHEYWMRHALTLAKRARDEREVPVGAVLVLNNRVIGVGWNRAIGLHDPTAHAEIMALRQGGLVMQNYRLIDAALYVTFEPCIMCAGAMIHSRIGRVVFGVRNSKRGAAGSLMNVLNYPGMNHRVEITEGVLVDECAALLCDFYRMPRQVLNAQKKARSNINSGGSSGGSSGSETLGTREGAPPESSGGSSGGSAKNTITKTLKLRIVRPYNSAEVEKIVVDEKNNREKVALEKNKDKVKEACSEHLKVAAYCTTQVERSACLFCKARKLDDKFYQKLRGQFPDAVFWQEIGEIFRQLQKQAAEIYNQSLIELYYEIFIKGKGFANASSVEHYLSDVCYTRAAELFKNAAIASGLRGKVKSNFRLKELKNMKSGLPTTKSDNFPIPLVKQKGGQYTGFEVSSHNDDFIIKIPFGRWQVKKEIDKYRPWEKFDFEQVRKSPRPISLLLSTQRRKRNKGWSKDEGTEAEIRKVMNGDYQTSYIEVKRGSKIGEKSAWMLNLSIDVPKIDKGVDPSIIGGIDVGVKSPLVCAINNALSRYSISDNDLFHFNKKMFARRRILLRKNRHKRAGHGAKNKLKPITIMTEKSKRFRKKLIERWACEIADFFIKNKVGTVQMENLESMKRKEDSYFNVRLRGFWPYAEMQNKIEFKLKQYGIVVRKVAPNNTSKTCSKCGHLNNYFNFEYRKKNKFPHFKCEKCNFKEDADYNAALNISNPKLKSTKEEP

SEQ ID NO: 1952 - protein, 726 aa, synthetic construct
SEVEFSHEYWMRHALTLAKRARDEREVPVGAILVLNNRVIGEGWNRAIGLHDPTAHAEIMALRQGGLVMQNYRLIDATLYVTFEPCVMCAGAMIHSRIGRVVFGVRNSKHGAAGSLVNVLNYPGMNHRVEITEGILADECAALLCDFYRMPRQVFNARKKAQSSINPSGSSGGSSGSETPGTSESATPESSGGSSGSSAKNTITKTLKLRIVRPYNSAEVEKIVADEKNNREKIALEKNKDKVKEACSKHLKVASYCTTRVERNACLFCKARKLDDKFYQRLRGQFPDAVFWQELGEIFRQLQKQAAEIYNQSLIELYYEIFIKGKGFANASSVEHYLSDVCYTRAAELFKNAAIASGLRGKVKSNFRLKELKNMKSGLPTTKSDNFPIPLVKQKGGQYTGFEISSHNDDFIIRIPFGRWQVKKEIDKYRPWEKFDFEQVRKSPKPISLLLSTQRRKRNKGWSKDEGTEAEIRKVMNGDYQTSYIEVKRGSKIGEKSAWMLNLSIDVPKIDKGVDPRIIGGIDVGVKSPLVCAINNAFSRYSVSDNDLFHFNKKMFARRRILLKKNRHKRAGHGAKNKLKPITILTEKSVRFRKKLIERWACEIADFFIKNKVGTVQMENLESMKGKEDSYFNIRLRGFWPYAEMQNKIEFKLKQYGIEIRKVAPNNTSKTCSKCGHLNNYFNFEYRKKNKFPHFKCEKCNFKENADYNAALNISNPKLKSTKEEP

SEQ ID NO: 1953 - protein, 726 aa, synthetic construct
SEDEFSHEYWMRHALTLAKRARDGREVPVGAVLVLNNRVIGEGWNRAIGLHDPTAHAEIMALRQGGLVMQNYRLIDATLYVTFEPCVMCAGAMVHSRIGRVVFGVRNSKRGAAGSLMNVLDYPGMGHRVEITEGILADECAALLSDFYCMPRQVFNAQKRARPSINSGGSSGGSSGSETPGTSESATPESSGGGSSGSAKNTITKTLQLRIVRPYNSAEVEKIVADEKNSREKIALERNKDKVKEACSKHLKMASYCTTQVERNACLFCKARKLDDKFYQKLRGQFPDAVFWQELGGIFRQLQKQAAVIYNQSLIELYYEIFIKGKGITNASRVEHYLSDVCYTRAAELFKNAAIASGLRSKVRSNFRLKELKNMKSGLPTTKSDNFPIPLVKQKGGQYTGFEISSHNSDFIIKIPFGRWQVKEEIDKFRPWEKFDFEQVRKSPKPISLLLSTQRRKRNKGWSKDEGTEAEIEKVMNGDYQTSYIEVKRGSKTGEKSAWMLNLSIDVPKIDKGVDPSIIGGVDVGVKSPLVCAINNAFSRYSISDNDLFRFNKKMFARRRILLKKNRHKRAGHGAKNKLKPISILTGKSERFRKKLIERWACEIADFFIKNKVGTVQMENLESMKRKEDSYFNIRLRGFWPYAEMQNKIEFKLKQYGIEVRKVAPNNTSKTCSKCGHLNNYFNFEYRKKNKFPHFKCEKCNFKEDADYNAALNISNPKLKSSKEEP

SEQ ID NO: 1954 - protein, 726 aa, synthetic construct
SEVEFSHEYWMRHALTLAKRARDEREVPVGAILVLNNRVIGEGWNRAIGLHDPTAHAEIMALRQGGLVMQNYRLIDATLYVTFEPCVMCAGAMIHSRIGRVVFGVRNNKHGAAGSLVNVLNYPGMNHRVEITEGILADECAALLCDFYRMPRQVFNARKKAQSSISPGGSSGGSSGSETPGTSESVTPKSSGGSSGGSAKNTITKTLKLRIVRPYNSAEVEKIVADEKNNREKIALEKNKGKVKEACSKHLEVAAYCTTQVERNACLFCKARKLDDKFYQKLRGQFPDAVFWQELGEIFRQLQKQAAEIYNQSLIELYYEIFIKGKGFANASSVEHYLSDVCYTRAAELFKNAAIASGLRNKVKSNFRLKELRSMKSGLPTTKSDNFPIPLVRQKGGQYTGFEISNHNSDFIIKIPFGRWQEKEEIDKYRPWEKFDFEQVRRSPKPISLLLSTQRRKKNKGWSKDEGTEAEIRRVMNGDYQTSYIEVKRGSKIGEKSAWMLNLSIDVPKIDMGVDPSIIGGIDVGVKSPLVCAINNAFSRYSISDNDLFHFNKKMFARRRILLKKNRRRRAGHGAKNKLKPITILTEKSVRFRKKLIERWACEIADFFIKNKVGTVQMENLESMKRKEDSYFNIRLRGFWPYAEMQNKIEFKLKQYGIEIRRVAPNNTSRTCSKCGHLNNYFNFEYRKKSKFPHFKCEKCNFREDADYNAALNISNPKLKSTKEEP

SEQ ID NO: 1955 - protein, 726 aa, synthetic construct
SEVEFSHEYWMRHALTLAKRARDEREVPVGAVLVLNNRVIGEGWNRAIGLHDPTAHAEIMALRQGGLVMQNYRLTDATLYVTFEPCVMCAGAMIHSRIGRVVFGVRNSKRGAAGSLMNVLNYPGMNHCVEITEGILVDECAALLCDFYRMPRQVLNAQKKAQSSISSGGSSGGSSGSETPGASGSVTPKSSGGSSAGSAKDTITKTLKLRIVRPYNSAEVEKIVADEKNNREKIALEKNKDKVKEACSKHLKVAAYCTTQVERNACLFCKARKLDDKFYQKLRGQFPDAVFWQELGEIFRQLQKQAAEIYNQSLIELYYEILIKGKGFANASSVEHYLSDVCYTRAAELFKNAAIASGLRGKVKSNFRLKELKNMKSGLPTTKSDNFPIPLVKQKGGQYTGFEISSHNDDFIIKIPFGRWQVKKEIDKYRPWEKFDFEQVRKSPKPISLLLSTQRRKRNKGWSKDEGTEAEIRKVMNGDYQTSYIEVKRGSKIGEKSAWMLNLSIDVPKIDKGVDPSIIGGIDVGVKSPLVCAINNAFSRHSISDNDLFHFNKKMFARRRILLKKNRHRRAGHGAKNKLKPIAVLAEKSEGFRKKLIERWACEVADFFIKNKVGTVQMENLESMKRREDSYFNIRLRGFWPYAEMQNKIEFKLKQYGIEIRKVAPNNTSKTCSRCGHLNDYFSFEFRKKNKFPRFKCEKCSFKENADYNAALNISNPKLKSTKEEP

SEQ ID NO: 1956 - protein, 726 aa, synthetic construct
SEVEFSHEYWMRHALTLAKRARDEREVPVGAVLVLNNRVIGEGWNRAIGLHDPTAHAEIMALRQGGLVMQNYRLIDATLYVTFEPCVMCAGAMIHSRIGRVVFGVRNSKRGAAGSLMNVLNYPGMNHRVGITEGILADECAALLCDFYCMPRQVLNAQKKARSCINPGGSSGGSRGSETPGTSESATPESSGGSSGGSAKNTITKTLKLRIVRPYNSAEVEKIVADEKDNRERIALEKSKGKVKEACSKHLKVASYCTTQVERNACLFCKARKLDDKFYQKLRGQFPDAVFWQELGEIFRQLQKQAAEIYNQSLIELYYVIFIKGKGLANASSVEHYLSDVCYTRAAELFKNAAIASGLRGKVKSNFKLKELKSMKSGLPSTKSDNFPIPLVKQRGGQYTGFEISSHNDDFIIKIPFGRWQAKKEIDKYRPWEKFDFEQVRKSPKPISLLLSTQRRKRNKGWGKDEGTEAEIKKVMNGDYQTSYIEVRRGSKIGEKSAWMLSLSIDVPKIDKGVDPSIIGGIDVGVKSPLVCAINNAFSRYSISDNDLFRFNKKMFARRRILLKKNRHKRAGHGAKNKLKPITILTEKSVRFRKKLIERWACEIADFFIKNKVGTVQMENLESMKRKEDSYFNIRLRGLWPYAEMQNKIEFKLKQYGIEIRKVAPNNTSKTCSKCGHLNNYFNFEYRKKNKFPHFKCEKCSFKENADYNAALNISNPKLKSTKVEP

SEQ ID NO: 1957 - protein, 726 aa, synthetic construct
SEVEFSHEYWMRHALTLAKRARDGREVPVGAVLVLNNRVIGEGWNRAIGLHDPTAHAEIMALRQGGLVMQNYRLIDATLYVTFEPCVMCAGAMIHSRIGRVVFGVRNNKHGAAGSLVNVLNYPGMNHRVEITEGILAGECAALLCDFYRMPRQVFNARKKAQSTINSGGSSGGSSSSETPGTSGSATPEDSGGGSGGSAKNTITKTLQLRIVRPYNSAEVEKIVADEKNNREKIALEKNKDKVREACSKHLKVASYCTTQVERNACLFCKARRLDDKFYQKLRGQFPDAVFWQEIGEIFRQLQKQAAEIYNQSLVELYYEVLIKGKGIANASSVEHYLSDVCYTRAAELFKNAAIASGLRNKIKSNFRLKELKNMKSGLPTTKSDNFPIPLVRQKGGKYTGFEISNHNGDFIIKIPFGRWQVKKEISKHRPWEKFDFEQVRKSPKPISLLLSTQRRKRNKGWGKDEGTEAEIRKVMNGDYQTSYIEVKRGSKIGEKSAWMLNLSIDVPKIDKGVDPSIIGGIDVGVKSPLVCAINNAFGRYSISDNDLFHFNKKMFARRRILLKKNRHKRAGHGAKNKLKPITILTEKSKRFRKKLIERWACEIADFFIKNKVGTVQMENLESMKRKEDSYFNIRLRGFWPYAEMQNKIEFKLKQYGIEIRKVAPNNTSKTCSKCGHLNDYFNFEYRKKNKFPHFKCEKCNFKENADYNAALNISNPKLKSTKKEP

SEQ ID NO: 1958 - protein, 726 aa, synthetic construct
SEVEFSHEYWMRHALTLAKRARDEREVPVGAVLVLNNRVIGEGWNRAIGLHDPTAHAEIMALRQGGLVMQNHRLVDATLYVTFEPCVLCAGAMVHSRIGRVVFGVRNSKRGAAGSLMNVLNYPGMNHRVEITEGILADECAALLCDFYRMPRQVFNARKKARSNINPGGSSGGSGGSETPGTSESPTPESSGGSSGGSAKNTITKTLQLRIVRPYNSAEVEKVVADEKNNREKIALEKNKDKVKEACSKHLKVASYCTTQVERNACPFCKARKLDDKFYQKLRGQFPDAVFWQELGEILRQLQKQAAEIYNQSLIELYYEIFIKGRGFANASSVEHYLSDVCYTRAAELFKNAAIASGLRGKVKSNFRLKELKNMKSGLPTTKSDNFPIPLVKQKGGQYTGFEISSHNDDFIIKIPFGRWQVKKEIDRYRPWEKFDFEQVRKSPKPISLLLSTQRRKRNKGWSKDEGTEAEIKKVMNGDYQISYIEVKRGSKIGEKSAWTLNLSVDVPKIDKGVDPSIIGGIDVGVKSPLVCAINNALSRYSISDNDLFHFNKKVFARRRILLKKNRHRRAGHGAKNKLKPITILTEKSKRFRKKLIERWACEIADFFIKNKVGTVQMENLESMKRKEDSYFNIRLRGFWPYAEMQNKIEFKLKQYGIKIRKVAPNNTSKTCSKCGHLSNYFSFEYRKKNKFPHFKCEKCNFKEDADYNAALNISNPKLKSTKEEP

SEQ ID NO: 1959 - protein, 726 aa, synthetic construct
SEVGFSHEYWMRHALTLAKRARDEREVPVGAVLVLNNRVIGEGWNRTTGLHDPTAHAEIMALRQGGLVTQNHRLVDATLYVTFEPCVMCAGAMVHSRIGRVVFGVRNSKRGAAGSLMNVLDYPGMGHRVEITEGILADECAALLCDFYCMPRQVFNAQKRAQSSINSGGSSGGSSGSDTPGTSESATPESSGGGSSGSAKNTITKTLQLRIVRPYNSAEVEKIVADEKNNREKIALEKNKDKVREACSKHLKVASYCTTQVERNACPFCKARKLDDRFYQKLRGQFPDAVFWQELGEILRQLQKQAAEIYNQSLIELYYEIFIKGRGFANASSVEHYLSDVCYTRAAELFKNAAIASGLRGKVKGNFRLKELKSMKSGLPTTKSDNFPIPLVKQKGGQYTGFEISSHNDDFIIKIPFGRWRAKKEIDKYRPWEKFDFEQVRKSPKPISLLLSTQRRKKNRGWSKDEGTEAEIKKVMNGDYQTSYIEVKRGSKIGEKSAWMLNLSIDVPKIDKGVDPSIIGGIDVGVKSPLVCAISNAFSRYSISDNDLFHFNKKMFARRRILLKKSKHKRAGHGAKNKLKPITILTEKSRRFRKKLIERWACEIADFFIKNKVGTVQMENLGSMKRKEDSYFNIRLRGFWPYAEMQNKIEFKLKQYGIEIRKVAPDNTSKTCSKCGHLNNYFNFEYRKKNKFPHFKCEKCNFKEDADYNAALNISNPKLKSTKEEP

SEQ ID NO: 1960 - protein, 726 aa, synthetic construct
SEVEFSHEYWMRHALTLAKRARDEREVPVGAVLVLNNRVIGEGWNRAIGLHDPTAHAEIMALRQGGLAMQNYRLVDATLYVTFEPCVLCAGAMVHSRIGRVVFGVRNSKRGAAGSLMNVLNHPGMNHRVEITGGILADECAALLCDFYCMPRQVFNAQKRAQSSINSGGSSDGSSGSETPGTSESATPESSGGSSGGSAKNTTTKTLKLRIVRPYNSAEVEKIVADEKNNREKIALEKNKDKVKEACSKHLKVAAYCTTQVERNACLFCKARKLDDKFYQKLRGQFPDAVFWQELGEIFRQLQKQAAEIYNQSLIELYYEIFIKGKGFANASSVEHYLSDVCYTRAAELFKNAAIASGLRGKVKSNFRLKELKNMKSGLPTTKSDNFPIPLVKQKGGQYTGFEISSHNSDFIIKIPFGRWQEKEEIDKYRPWEKFDFEQVRRSPKPISLLLSTQRRKKNKGWSKDEGTEAEIRKVMNGDYQTSYIEVKRGSKIGEKSAWMLNLSIDVPKIDKGVDPSIIGGIDVGVKSPLVCAINNAFSRYSISDNDLFHFNKKMFARRRILLKKNRHKRAGHGAKNKLKPITIMTEKSKRFRKKLIERWACEIADFFIKNKVGTVQMENLESMKRKEDSYFNIRLRGFWPYAEMQNKIEFKLKQYGIVVRKVAPNNTSKTCSQCGHLNNYFNFEYRKKNKFPYFKCEKCNFKENADYNAALNISNPQLKCTKGEP

SEQ ID NO: 1961 - protein, 726 aa, synthetic construct
SEVEFSHEYWMRHALALAKRARDEREVPVGAILVLNNRVIGEGWNRAIGLHDPTAHAEIMALRQGGLVMQNYRLIDATLYVTFEPCVMCAGAMIHSRIGRVVFGVRNNKHGAAGSLVNVLNYPGMNHRVEITEGILADECAALLCDYYRMPRQVFSARKKAQSSINSGGSSDGGSGSETPGTCESVTPESSGGSSGGSAKNTITKTLQLRIVRPYNSAEVEKIVADEKNNREKIALEKNKDKVKEACSKHLKVASYCTTQVERNACLFCKARKLDDKFYQKLRGQFPDAVFWQELGEIFRQLQKQAAEIYNQSLIELYYVIFIKGKGLANASSVEHYLSDVCYTRAAELFKNAAIASGLRGKVKSNFKLKELKSMKSGLPSTKSDNFPIPLVKQKGGQYTGFEISSHNDDFIIKIPFGRWQAKKEIDKYRPWEKFDFEQVRKSPKPISLLLSTQRRKRNKGWSKDEGTEAEIKKVMNGDYQTSYIEVKRGSKIGEKSAWMLSLSIDVPKIDKGVDPSIIGGIDVGVKSPLVCAINNAFSRYSISDNDLFHFNKKMFARRRILLKKNRRRRAGHGAKNKLKPITILTEKSARFRKKLIERWACEIADFFIKNKVGTVQMENLESMKRKEDSYFNIRLRGFWPYAEMQNKIEFKLKQYGIEIRRVAPNNTSRTCSKCGHLNNYFNFEYRRKYKFPHFKCEKCNFKEDADYNAALNISNPKLKSTKEEP

SEQ ID NO: 1962 - protein, 726 aa, synthetic construct
SEVEFSHEYWMRHALTLAKRARDEREVPVGAVLVLNNRVIGVGWNRAIGLHDPTAHAEIMALRQGGLVMQNYRLTDATLYVTFEPCVMCAGAMIHSRIGRVVFGVRNSKRGAAGSLMNVLNYPGMNHCVEITEGILVDECAALLCDFYRMPRQVLNAQKKAQSSISSGGSSGGSSCSETPGASESVTPKSSGGGSAGSTKNTITKTLQLRIVRPYNSAEVEKIVADEKNNREKIALEKNKDKVKEACSKHLKVAAYCTTRVERNACPFCRARKLDDKFYQKLGGQFPDAVFWQELGEVFRQLQRQAAEIYNRSLIELYYEIFIKGKGFANASSVEHYLSDVCYTRAAELFKNAAIASGLRGKVKSNFRLKELKNMKSGLPTTKSDNFPIPLVKQKGGQYTGFEISSHNDDFIIKIPFGRWQAKKEIDKYRPWERFDFEQVRKSPKPISLLLSTQRRKRNKGWSKDEGTEAEIRKVMNGDYQTSYIEVKRGSKIGEKSAWMLNLSIDVPKIDKGVDPSIIGGIDVGVKSPLVCAINNAFSRYSISDNDLFHFNKKMFARRRILLKKNRHRRAGHGAKNKLKPITILTEKSVRFRKKLIERWACEIADFFIKNKVGTVQMENLESMKRKEDSYFNIRLRGFWPYAEMQNKIEFKLKQYGIEIRRVAPNNTSRTCSKCGHLNNYFNFEYRKKNKFPHFKCEKCNFKENADYNAALNISNPRLKSTREEP

SEQ ID NO: 1963 - protein, 726 aa, synthetic construct
SEVEFSHEYWMRHALTLAKRARDEREVPVGAILVLNNRVIGVGWNRAIGLHDPTAHAEIMALRQGGLVLQNYRLIDATLYVTFEPCVMCAGAMIHSRIGRVVFGVRNNKHGAAGSLVNVLNYPGMNHRVEITEGILANECAALLCDFYRMPRQVFNARKKAQSSINSGGSSGGSSGSETPSTSESATPESSGGSSGSSAKNTITKTLQLRIVRPYNSAEVEKIVADEKNNREKIALEKNKDKVKEACSKHLKVASYCTTQVERNACLFCKARKLDDKFYQRLRGQFPDAVFWQELGEIFRQLQKQAAEIYNQSLIELYYEIFIKGKGFANASSVEHYLSDVCYTRAAELFKNAAIASGLRGKVKSNFRLKELKNMKSGLPTTKSDNFPIPLVRQKGGQYTGFEISSHNDDFIIKIPFGRWQAKKEIDKYRPWEKFDFEQVRKNPKPISLLLSTQRRKRNKGWSKDEGTEAEIRKVMNGDYQTSYIEVKRGSKIGEKSAWMLNLSIDVPKIDKGVDPSIIGGIDVGVKSPLVCAINNAFSRYSISDNDLFRFNKKVFARRRILLKKNRHKRAGHGTKNKLKPITILAEKSGRFRKKLIERWACEIANFFIKNKVGTVQMENLEGMKRKEDSYFNIRLRGFWPYAEMQNKIEFKLKQYGIKIRKVAPNNTSKTCSKCGHLNNYFSFEYRKKNKFPHFKCEKCNFREDADYNAALNISNPKLKSTKEDP

SEQ ID NO: 1964 - protein, 726 aa, synthetic construct
SEVEFSHEYWMRHALTLAKRARDEREVPVGAVLVLNNRVIGEGWNRAIGLHDPTAHAEIMALRQGGLVLQNYRLVDATLYVTFEPCVMCAGAMIHSRVGRVVFGVRNSKHGAAGSLMNVLNYPGMNHRVEITEGILADECAALLCDFYRMPRRVFNARKKAQPSIDPGGPSGGSSGSETPGTSESATPESSGGSSGGSAKNTITKTLKLRIVRPYNGAEVEKIVTDEKNNREKIALEKNKDKVKEACSKHLKMASYCTTQVERNACLFCKARKLDDKFYQKLRGQFPDAVFWQELGEIFRQLQKQAAEIYNQSLIELYYEIFIKGKGFANASSVEHYLSDVCYTRAAELFKNAAIASGLRGKVKSNFRLKELKNMKSGLPTTKSDNFPIPLVKQKGGQYTGFEISSHNDDFIIKIPFGRWQAKKEIDKYRPWEKFDFEQVRKSPKPISLLLSTQRRKRNKGWSKDEGTEAEIRKVMNGDYQTSYIEVKRGSKIGEKSAWMLNLSIDVPKIDKGVDPSIIGGIDVGVKSPLVCAINNAFSRYSISDNDLFHFNKKMFARRRILLKKSRHKRAGHGAKNKLKPISILTEKSERFRKKLIERWACEIANFFIKNKVGTVQMENLESMKRKEDSYFNIRLRGFWPYAEMQNKIEFKLKQYGIEIRKVAPNNTSKTCSKCGHLNNYFNFEYRKKNKFPHFKCEKCNFKENADYNAALNISNPKLKSTKEEP

SEQ ID NO: 1965 - protein, 726 aa, synthetic construct
SEVEFSHEYWMRHALTLAKRARGEREVPVGAVLVLNNRVIGEGWNRAIGLHDPTAHAEIMALRQGGLVMQNYRLTDATLYVTFEPCVMCAGAMIHSRIGRVVFGVRNNKHGAAGSLVNVLNYPGMNHRVEITEGILADECTALLCDFYRMPRQVFNARKKAQSSISPDGSSGGSSGSETPGTSESATPESSGGSSGGSAKNTITKTLKLRIVRPYNSAEVEKIVADEKNNREKIALEENKDKVKEACSKHLKVAAYCTTQVERNACLFCKARRLDDKFYQKLRGQFPDAVFWQEIGEIFRQLQKQAAEIYNQSLIELYYEIFIKGKGIASASRVGHYLSDVCYTRAAELFKNAAIASGLRSKIKSNFRLKELKNMKSGLPTTKSDNFPIPLVKQKGGQYTGFEISNHNSDFIIKIPFGRWQVKREIDKYRPWEKFDFEQVRKSPKPISLLLSTQGRRRNKGWSKDEGTEAEIKKVMNGDYQTSYIEVKRGSKTGEKSAWMLNLSIDVPKIDKGVDPCIIGGIDVGVKSPLVCAINGAFSRYSISDNDLFHFNKRMFARRRILLKKNGHKRAGHGAKNKLKPITIMTEKSKRFRKKLIERWACEIADFFVKNKVGTVQMENLESMKRKEDSYFNIRLRGFWPYAEMQNKIEFKLKQYGIEIRKVAPNNTSRTCSKCGHLNNYFDFEYRKKNKFPHFKCEKCNFKENADYNAALNISNPKLKSTKEEP

SEQ ID NO: 1966 - protein, 726 aa, synthetic construct
SEVEFSHEYWMRHALTLAKRARDEREVPVGAVLVLNNRAIGEGWNRAIGLHDPTAHAEIMALRQGGLVMQNYRLTDATLYVTFEPCVMCAGAMIHSRIGRVVFGVRNSKRGAAGSLMNVLNYPGMNHCVEITEGILVDECAALLCDFYRMPRQVLNAQKKAQSSISSGGSSGGSSGSETPGNSESATPESSGGSSGGSAKNTITKTLKLRIVRPFNSAEVERIVADEKNNREKIALEKNKDKVKEACSEHLKVAAYCTTQVERSACLFCKARKLDDKFYQKLRGQFPDAVFWQEIGEIFRQLQKQAAEIYNQSLIELYYEIFIKGRGFANASSVEHYLSDVCYTRAAELFKNAAIASGLRGKVKSNFRLKELKNMKSSLPTTKSDNFPIPLVKQKGGQYTGFEISSHNDDFIIKIPFGRWQVKKEIDKYRPWEKFDFEQVRKSPKPISLLLSTQRRKRNKGWGKDEGTEAEIRKVMNGDYQTSYIEVKRGSKTGEKSAWMLNLSIDVPKIDKGVDPSIIGGIDVGVKSPLVCAINNAFSRYSISDNDLFRFNKKMFARRRILLKKNRHKRAGHGAKNKLKPITILTEKSVRFRKKLIERWACEIADFFVKNKVGTVQMENLESMKRKEDSYFNIRLRGFWPYAEMQNKIEFKLKQYGIEIRKVAPNNTSKTCSECGHLNNYFNFEYRKKNKFPHFKCEKCSFRENADYNAALNISNPKLKSTKEEP

SEQ ID NO: 1967 - protein, 726 aa, synthetic construct
SEVEFSHEYWMRHALTLAKRARDEREVPVGAILVLNNRVVGEGWNRAIGLHDPTAHAEIMALRQGGLVMQNYRLTDATLYVTFEPCVMCAGAMIHSRIGRVVFGVRNNKHGAAGSLVNVLNYPGMNHRVEITEGILADECAALLCDFYRMPRQVFNARKKAQSSINPGGSSGGSNGSETPGTSESATPESSGGSSGGSAKNTITKTLKLRIVRPYNSAEVEKIVADEKNNREKIALERNKDRVKEACSKHLKVAAYCTTQVERNACLFCKARRLDDMFYQKLRGQFPDAVFWQETGEIFRQLQRQAAEIYNQSLIELYYEIFIKGKGFANASSVEHYLSDVCYTRAAELFKNAAIASGLRGKVKSNFRLKELKNMKSGLPTTKSDNFPIPLVKQKGGQYTGFEISSHNDDFIIKIPFGRWQVKKEIDKYRPWEKFDFEQVRKSPKPISLLLSTQRRKRNKGWGKDGGTEAEIRKVMNGDYQTSYIEVKRGSKTGEKSAWMLNLSIDVPKIDKGVDPSIIGGIDVGVKSPLVCAINNAFSRYSISDNDLFRFNKKMFARRRILLKKNRHKRAGHGVKNKLKPISILTGKSERFRKKLIERWACEIADFFIKNKVGTVQMENLESMKRKEDSYFNIRLRGFWPYAEMQNKIEFKLKQYGIEIRKVAPNNTSKTCSKCGHLNNYFNFEYRKKNKFPHFKCEKCNFKENADYNAALNISNPKLKSTKGEP

SEQ ID NO: 1968 - protein, 726 aa, synthetic construct
SEVEFSHEYWMRHALTLAKRARDEREVPVGAILVLNNRVIGEGWNRAIGLHDPTAHAEIMALRQGGLVMQNYRLTDATLYVTFEPCVMCAGAMIHSRIGRVVFGVRNSKRGAAGSLMNVLNYPGMNHCVEITEGILVDECAELLCDFYRMPRQVLNARKKAQSSINSGGSSDGGSSSETPGTSESATPESSGGSSGGSAKNTITKTLKLRIVRPYNSAEVEKIVADEKNNREKIALEKNKDKVKEACSEHLKVAAYCTTQVERSACLFCKARELDGKFYQKLRGQFPDAVFWQELGEIFRQLQKQAAEIYNQSLIELYYEIFVKGKGIANTSRMEHYLSDVCYTRAAGLFKNAAIASGLRGKIKSNFRLKELKSMKSGLPTTRSDNFPIPLVKQKGGQYTGFEISNHDSDFIIKIPFGRWQVKKEIDKYRPWEKFDFEQVRKSPKPISLLLSTQRRKRNKGWSKDEGTEAEIKKVMNGDYQTSYIEVKRGSKIGEKSAWMLNLSIDVPKIDKGVDPSIIGGIDVGVKSPLVCAINNAFSRYSISDNDLFHFNKKMFARRRILLKKNRHKRAGHGAKNKLKPLTILTGKSKRFRKKLIERWACEIADFFIKNKVGTVQMENLESMKRKEDSYFNIRLRGFWPYAEMQNKIEFKLKQYGIEIRRVAPNNTSKTCSKCGHLNNYFNFEYRKRNKFPHFKCEKCNFKENADYNAALNISNPKLKSPKEES

SEQ ID NO: 1969 - protein, 726 aa, synthetic construct
SEDEFSHEYWMRHALTLAKRARDGREVPVGAVLVLNNRVIGEGWNRAIGLHDPTAHAEIMALRQGGLVMQNYRLIDATLYVTFEPCVMCAGAMVHSRIGRVVFGVRNSKRGAAGSLMNVLDYPGMGHRVEITEGILADECAALLCDFYCMPRQVFNAQKRAQSSINSGGSSGGSSGSETPGTNESATPESSGGGSSGSAKNTITKTLKLRIVRPYNSAEVEKIVADEKNNREKIALEKNKDKVKEACSKHLRVAAYCTTQVERNACLFCKARKLDDKFYQKLRGQFPDAVFWQELGEIFRQLQKQAAEIYNQSLIELYYEIFIKGKGFANASSVEHYLSDVCYTRAAELFKNAAIASGLRGKVKSNFRLKELKNMKSGLPTTKSDNFPIPLVKQKGGQYTGFEISSHNDDFIIKIPFGRWQVRKEIDKYRPWEKFNFEQVRKSPKPISLLLSTQRRKRNKGWSKDEGTEAEIRKVMNGDYQTSYIEVKRGSKIGEKSAWMLSLSIDVPKIDKGVDPSIIGGIDVGVKSPLVCAINNAFNRYSISDNSLFHFNKKMFARRRILLKENRLKRAGHGAKNKLKPISILTEKSERFRKKLIERWACEIANFFIKNKVGTVQMENLESMRRKEDSYFNIRLRGFWPYAEMQNKIEFKLKQYGIEIRKVAPNNTSKTCSKCGHLNNYFNFEYRKKNKFPHFKCEKCNFKENADYNAALNISNPKLKSTKEEP

SEQ ID NO: 1970 - protein, 726 aa, synthetic construct
SEVEFSHEYWMRHALTLAKRARDEREVPVGAILVLNNCVIGEGWNRAIGLHDPTAHAEIMALRQGGLVMQNYRLIDATLYVTFEPCVMCAGAMIHSRIGHVVFGVRNNKHGAAGSLVNVLDYPGMNHRVEITEGILADECAALLCDFYRMPRQVLNARKKAQSSISPGGSSGSSSGSETPGTSESATPESSGGSSGGSAKNTITKTLKLRIVRPYNSAEVEKIVADEKDNREKIALEKNKDKVKEACSKHLKVAAYCTTQVERNACLFCRARKLDDKFYQKLRGQFPDAVFWQEIGEIFRQLQKQAAEIYNQSLIELYYEIFIKGKGFANASSVEHYLSDVCYTRAAELFKNAAIASGLRNKIKSNFRLKELRNMKSGLPTTKSDNFPIPLVRQKGGQYTGFEISSHNDDFIIKIPFGRWQAKKEIDKYRPWEKFDFEQVRKSPKPISLLLSTQRRKRNKGWSKDEGTEAEIRRVMNGDYQTSYIEVKRGSKIGEKGAWMLNLSIDVPKVDKGVDPSIIGGIDVGVKSPLVCAINNAFSRYSISDNDLFRFNKKMFARRRILLKKNRHQRAGHGAKNKLKPITILTEKSGRFRKKLIERWACEIADFFIKNKVGTVQMENLESMKRKEDSYFNIRLRGFWPYAEMQNRIEFKLKQYGIKIRRVAPNNTSKTCSKCGHLNNYFSFEYRKKNKFPHFKCEKCNFKEDADYNAALNISNPKLKSTKEEP

SEQ ID NO: 1971 - protein, 726 aa, synthetic construct
SEVEFSHEYWMRHALTLAKRARDEREVPVGAVLVLNNRVIGEGWNRTTGLHDPTAHAEIMALRQGGLVMQNHRLVDATLYVTFEPCVMCAGAMIHSRISRVVFGVRNSKRGAAGSLTNVLNYPGMNHRVEITEGILVDECAALLCDFYRMPRQVFSAQKKAQSTINSGGSSGGSSGSETPGTSESPTPESSGGSSGGSAKNTITKTLKLRIVRPYNSAEVEKIVAEEKDNREKIALEKNKDKVKEACSKHLKVASYCTTQVERNACPFCKARKLDDKFYQKLRGQFPDAVFWQELGEILRQLQKQAAEIYNQSLIELYYEVFIKGKGFANASSVEHYLSDVCYTRAAELFKNAAIASGLRGKVKSNFRLKELKNMKSGLPTTKSDNFPIPLVKQKGGQYTGFEISSHNDDFIIKIPFGRWQVKKEIDKYRPWEKFDFEQVRKSPKPISLLLSTRRRRRNKGWSKDEGTEAEIRKVMNGDYQTSYIEVKRGSKIGEKSAWMLSLSIDVPKIDKGVDPSIIGGIDVGVKSPLVCAINNALSRYSISDNDLFHFNKKMFARRRILLKKNRHRRAGHGAKNKLKPIAVLAEKSEGFRKKLIERWACEVADFFIKNKVGTVQMENLESMKRREDSYFNIRLRGFWPYAEMQNKIEFKLRQYGIEIRKVAPNNTSKTCSKCGHLNNYFDFEYRKKNKFPHFKCEKCNFKENADYNAALNISNPKLKSTKEEP

SEQ ID NO: 1972 - protein, 726 aa, synthetic construct
SEVEFSHEYWMRHALTLAKRARDEREVPVGAILVLNNRVIGEGWNRAIGLHDPTAHAEIMALRQGGLVMQNYRLIDATLYVTFEPCVMCAGAMIHSRIGRVVFGVRNNKHGAAGSLVNVLDYPGMNHRVEITEGILADECAALLCDFYRMPRQVFNARKRAQSSINSGGSSGGSSGSETPGTSESATPESSGGGSSGSAKNTITKTLQLRIVRPYNSAEVEKIVADEKNNREKIALEKNKDKVREACSKHLKVASYCTTQVERNACPFCKARKLDDKFYQKLRGQFPDAVFWQELGEILRQLQKQAAEIYNQSLIELYYEIFIKGKGFANASSVEHYLSDVCYTRAAELFKNAAIASGLRGKVKSNFRLKELKNMKSGLPTTKSDNFPIPLVKQKGGQYTGFEISNRNSDFIIKIPFGRWQVKKEINKYRPWEKFDFEQVRKSPKPISLLLSTQRRKRNKGWSKDEGTEAEIRKVMNGDYQTSYIEVKRGSRIGEKSAWMLSLSIDVPKIDRGVDPSIIGGIDVGVKSPLVCAINNALSRYSISDNDLFHFNKKMFARRRILLKKNRHRRAGHGARNKLKPITVLTEKSKRFRKKLIERWACEIANFFIKNKVGTVQMENLESMKRKEDSYFNIRLRGLWPYAEMQNKIEFKLKQYGIEIRKVAPNNTSKTCSKCGHLNNYFNFEYRKRNKFPHFKCEKCNFKENADYNAALNISNPKLKGTKEEP

SEQ ID NO: 1973 - protein, 726 aa, synthetic construct; identical to SEQ ID NO: 684

SEQ ID NO: 1974 - protein, 726 aa, synthetic construct
SEVEFSHEYWMRHALTLAKRARDEREVPVGAVLVLNNRVIGGGWNRAIGLHDPTAHAEIMALRQGGLVMQNCRLVDATLYVTFEPCVMCAGAMIHSRIGRVVFGVRNSKRGAAGSLMNVLNYPGMNHRVEITEGILADECAALLCDFYRMPRQVFDAQKKARSNINSGGSSGGSSGSETPGASGSVIPKSSGGSSAGSTKDTITKTLKLRIVRPYNSAEVEKVVADEKNNREKIAMEKNKDKVKEACSKHLKVASYCTTQVERNACLFCKARKLDDKFYQKLRGQFPDAVFWQELGGIFRQLQKQAAEIYNQSLIELYYEIFIKGKGITNASRVEHYLSDVCYTRAAELFKNAAIASGLRSKVRSNFRLKELKNMKSGLPTTKSDNFPIPLVKQKGGQYTGFEISSHNDDFIIKIPFGRWQVKKEIDKYRPWEKFDFEQVRKSPKPISLLLSTRRRKRNKGWSKDEGTEAEIRKVMNGDYQTSYIEVRRGSKIGEKSAWMLNLSIDVPKIDKGVDPSIIGGIDVGVKSPLVCAINNAFSRYSISDNELFHFNKKMFARRRILLKKNRHKRAGHGAKNKLKPISILTEKSERFRKKLIEKWACEIADFFIKNKVGTVQMENLESMKRKEDSYFNIRLRGFWPYAEMQNKIEFKLKQYGIVIRKVAPNNTSRTCSKCGHLNNYFNFEYRKKNKFPHFKCEKCNFKENADYNAALNISNPKLKSTKEEP

SEQ ID NO: 1975 - protein, 726 aa, synthetic construct
SGVEFSHEYWMRHALTLAKRACDEREVPVGAVLVLNNRVIGEGWNRAIGLHDPTAHAEIMALRQGGLVMQNYRLIDATLYVTFEPCVMCAGAMIHSRIGRVVFGVRNSKHGAAGSLVNVLNYPGMNHRVEITEGILADECAALLCDFYRMPRQVFNARKKAQSSINPSGSSGGSSGSVTPGTSESPTPESSGGSPGGSAKNTITKTLKLRIVRPYNSAEVEKIVADEKNNREKIALEKNKDKVKEACSKHLKVAAYCTTQVERSACLFCKARKLDDKFYQKLRGQFPDAVFWQEVGEIFRQLQKQAAEIYNQSLIELYYEIFIKGKGFANASSVEHYLSDVCYTRAAELFKNAAIASGLRGKVKSNFRLKELKNMKSGLPTTKSDNFPIPLVKQKGGQYTGFEISSHNDDFIIKIPFGRWQVKKEIDKYRPWEKFDFEQVRKSPKPISLLLSTQRRKKNRGWSKDEGTEAEIKKVMNGDYQTSYIEVKRGSKIGEKSAWMLNLSIDVPKIDKGVDPSIIGGIDVGVKSPLVCAINNAFSRYSISDNDLFHFNKKMFARRRILLKKNRHKRAGHGAKNKLKPISILTEKGERFRKKLIERWACEIANFFIKNKVGTVQMENLESMKRKEDSYFNIRLRGFWPYAEMQDKIEFKLKQYGIEIRKVAPNNTSKTCSRCGHLNNYFNFEYRKKNKFPHFKCEKCSFKENADYNAALNISNPKLKSTKEEP

SEQ ID NO: 1976 - protein, 726 aa, synthetic construct
SEVEFSHEYWMRRALTLAKRARDEREVPVGAVLVLNNRVIGVGWNRAVGLHDPTAHAEIMALRQGGLVMQNYRLIEATLYVTFEPCIMCAGAMIHSRIGRVVFGVRNSKRGAAGSLMNVLNYPGMNHRVEITEGILADECAALLCDYYRMPRQVFNARKKAQSSINSGGSFDGGSGSETPGTSESATPESSGGSSGGSAKNTITKTLKLRIVRPYNSAEVEKIVADEKNNREKIALEKNKDKVKEACSEHLKVAAYCTTQVERSACLFCKARKLDDKFYQKLRGQFPDAVFWQELGEIFRQLQKQAAEIYNQSLIELYYEIFIKGKGFANASSVEHYLSDVCYTRAAELFKNAAIASGLRGKVKSNFRLKELKNMRSGLPTTKSDNFPIPLVKQKGGQYTGFEISGHNGDFIIKIPFGRWQVKKEIDKYRPWEKFDFEQVRKSPKPISLLLSTRRRKRNKGWSKDEGTEAEIRKVMNGDYQTSYIEVKRGGKTGEKSAWMLSLSIDVPKIDRGVDPSIIGGIDVGVKSPLVCAINNAFSRYSISDNDLFRFNKKMFARRRILLKKNRHKRAGHGAKNKLKPISILTGKSERFRKKLIERWACEIADFFIKNKVGTVQMENLEGMKRKEDSYFNIRLKGFWPYAEMQNKIEFKLKQYGIEIRKVAPNNTSKTCSKCGHLNNYFNFEYRKKNKFPHFKCEKCNFKENADYNAALNISNPKLKSTKEEP

SEQ ID NO: 1977 - protein, 726 aa, synthetic construct
SEVEFSHEYWMRHALTLAKRARDEREVPVGAVLVLNNRVIGEGWNRAIGLHDPTAHAEIMALRQGGLVMQNYRLVDATLYVTFEPCVLCAGAMVHSRIGRVVFGVRNSKRGAAGSLMNVLNYPGMNHRVEITEGILADECAALLCDFYRMPRRVFNAQKKARSNINSGGSSGGGSGSETPSTSESTTPESSGGSSGGPAKNTITKTLKLRIVRPYNSAEVEKIVADEKNNREKTALEKNKDKVKEACSKHLKVAAYCTTQVERNACLFCKARKLDDEFYQKLRGQFPDAVFWQEVGEIFRQLQKQAAEIYNQSLIELYYEIFIKGEGFANASSVEHYLSDVCYTRAAELFKNAAIASGLRGKVKSNFRLKELKNMKSGLPTTKSDNFPIPLVKQKGGQYTGFEISNHNSDFIIKIPFGRWQVKKEINKYRPWEKFDFEQVRKSPKPISLLLSTQRRKRNKGWSKDEGTEAEIEKVMNGDYQTSYIEVKRGSKIGEKSAWMLSLSIDVPKIDKGVDPSIIGGIDVGVKSPLVCAINNAFGRHSISDNDLFHFNKKMFARRRILLKKNRHKRAGHGAKNKLKPITVLTEKSVRFRKKLIERWACEIADFFIKNKVGTVQMENLESMKRREDSYFNIRLRGFWPYAEMQNKIEFKLKQYGIKVRKVAPNNTSKTCSKCGHLNNYFSFEYRKKNKFPRFKCEKCNFKENADYNAALNISNPKLMSTKGEP

SEQ ID NO: 1978 - protein, 726 aa, synthetic construct
SEVEFSHEYWMRHALTLAKRARDEREVPVGAVLVLNNRVIGEGWNRAIGLHDPTAHAEIMALRQGGLVMQNYRLIDATLYVTFEPCVMCAGAMIHSRIGRVVFGVRNNKHGAAGSLVNVLNYPGMNHRVEITEGILANECAALLCDFYRMPRQVFNARKKAQSSINPGGSSGGSSGSETPGTSESATPESSGGSSGGSAKNTITKALKLRIVRPYNSAEVEKIVADEKNNRERIALEKNKDKVKEACSKHLKVAAYCTTQVERNACLFCKARKLDDEFYQKLRGQFPDAVFWQEIGEIFRQLQKQAAEIYNQSLIELYYEIFIKGRGFANASSVEHYLSDVCYTRAAELFKNAAIASGLRGKVKGNFRLKELKNMKSGLPTTKSDNFPIPLVKQKGGKYTGFEISSHNDDFIIRIPFGRWQVKKEIDKYRPWEKFDFEQVRKSPKPISLLLSTQRRKRNKGWSKDEGTEAEIRKVMNGDYQTSYIEVKRGSKIGEKSAWMLNLSIDVPKTDKGVDPSIIGGIDVGVKSPLVCAINNAFSRYSISDNDLFHFNKKMFARRRILLGKSRHKRAGHGTKNKLKPITILTEKSKRFRKKLIERWACEIADFFIKNKVGTVQMENLESMKRKEDSYFNIRLRGFWPYAEMQNKIEFKLKQYGIEIRKVAPNNTSRTCSKCGHLNNYFNFEYRKKNKFPHFKCEKCNFKEDADYNAALNISNPKLKSTKEEH

SEQ ID NO: 1979 - protein, 726 aa, synthetic construct
SEVEFSHEYWMRHALTLAKRARDEREVPVGAVLVLNNRVIGEGWNRAIGLHDPTAHAEIMALRQGGLVMQNYRLTDATLYVTFEPCVMCAGAMIHSRIGRVVFGVRNSKRGAAGSLMNVLNYPGMNHCVEITEGILVDECAALLCDFYRMPRQVLNAQKKAQSSISSGGSSGGSSCSETPGASESVTPKSSGGGSAGSTKNTITKTLKLRIVRPYNSAEVEKIVADEKNSREKIALEKNKDKVKEACSKHLKVAAYCTTQVERNACLFCKARRLDDKFYQKLRGQFPDAVFWQEIGEIFRQLQKQAAEIYNQSLVELYYEIFIKGKGFANASSVEHYLSDVCYTRAAELFKNAAIASGLRGKVKSNFRLKELKNMKSGLPTTKSDNFPIPLVKQKGGQYTGFEISSHNDDFIIKIPFGRWQVKKEIDKYRPWEKFDFEQVRKSPKPISLLLSTQRRKRNKGWSKDEGTEAEIRKVMNGDYQTSYIEVKRGSKIGEKSAWMLNLSIDVPKIDKGVDPSIIGGIDVGVKSPLVCAISNAFSRYSISDNDLFHFNKKMFARRRILLKKSKHKRAGHGAKNKLKPITILTEKSRRFRKKLIERWACEIANFFIKNKVGIVQMENLESMKRKEDSYFNIRLRGFWPYAEMQNKIEFKLKQYGIVVRKVAPNNTSKTCSKCGHLNNYFNFEYRKKNKFPHFKCEKCNFKENADYNAALNISNPKLKSTKEEP

SEQ ID NO: 1980 - protein, 726 aa, synthetic construct
SEVEFSHEYWMRHALTLAKRARDEREVPVGAVLVLNNRVIGVGWNRAIGLHDPTAHAEIMALRQGGLVMRNYRLIDATLYVTFEPCAMCAGAMIHSRIGSVVFGVRNSKRGAAGSLMNVLNYPGMNHRVEITEGILADECAALLCDFYRMPHQVLNAQKKAQSSINSGGSSGGSSGSETPGTSGSATPEGSGGSSGGFAKNTITKTLKLRIVRPYNSAEVEKIVADEKNNREKIALEKNKGKVKEACSKHLKVATYCTTQVERNACLFCKARKLDDKFYQKLRGQFPDAVFWQEVGEIFRQLQKQAAEIYNQSLIELYYEIFIKGKGIANASSVEHYLSDVCYTRAAELFKNAAIASGLRNKVKSNFRLKELRSMKSGLPTTKSDNFPIPLVKQKGGQYTGFEISSHNDDFIIKIPFGRWQAKKEIDKYRPWEKFDFEQVRRSPKPISLLLSTQRRKRNKGWSKDEGTEAEIRKVMNGDYQTSYIEVKRGSKIGEKSAWMLNLSIDVPKIDKGVDPSIIGGIDVGVKSPLVCAINNAFSRYSISDNDLFHFNKKMFARRRILLKKNRHKRAGHGARNKLKPITVLTEKSERFRKKLIERWACEIADFFVKNKVGTVQMENLESMKRREDSYFNIRLRGFWPYAKMQNKIEFKLKQYGIEIRKVAPSNTSKTCSKCGHLNNYFNFEYRKKNKFPHFKCEKCNFKENADYNAALNISSPKLKSTKEEP

SEQ ID NO: 1981 - protein, 726 aa, synthetic construct
SEVEFSHEYWMRRALTLAKRARDEREVPVGAVLVLNNRVIGVGWNRAIGLHDPTAHAEIMALRQGGLVTQNYRLIDATLYVTFEPCIMCAGAMIHSRIGRVVFGVRNSKRGAAGSLMNVLDYPGMNHRVEITEGILAGECAALLCDFYRMPRQVFNAQKKAQSNINPGGSSGGSGGGETPGTSESVTPKSSGGSSAGSTKDTITKTLKLRIVRPYNSAEVEKIVADEKNSREKIALEKNKDKVKEACSEHLKVAAYCTTQVERSACLFCKARKLDDRFYQKLRGQFPDAVFWQEISEIFRQLQKQAAEIYNQSLIELYYEILIKGKGIANASRVEHYLSDVCYTRAAELFKNAAIASGLRSKIKSNFRLKELRSMKSGLPTTKSDNFPIPLVKQKGGQCTGFEISNHNSDFIIKIPFGRWQVKKEIDKYRPWEKFDFEQVRKSPKPISLLLSTQRRRRNKGWSKDEGTEAEIRKVMNGDYQASYIEVKRGSKIGEKSAWMLSLSIDVPKIDKGVDPSIIGGIDVGVKSPLVCAINNAFGRYSISDNDLFRFNKKMFARRRILLKKNRHKRAGHGAKNKLKPISILTGKSERFRKKLIERWACEIADFFIKNKVGTVQMENLESMKRKEDSYFNIRLRGFWPYAEMQNKIEFKLKQYGIEIRKVAPNNTSKTCSKCGHLNNYFNFEYRKKNKFPHFKCEKCNFKENADYNAALNISNPKLKSTKEEP

SEQ ID NO: 1982 - protein, 726 aa, synthetic construct
SEVEFSHEYWMRHALTLAKRARDEREVPVGAVLVLNNRVIGEGWNRAIGLHDPTAHAEIMALRQGGLVMQNYRLIDATLYVTFEPCVMCAGAMVHSRIGRVVFGVRNSKRGAAGSLLNVLDHPGMDHRVEITEGILTDECATLLCDFYRMPRQVFNAQKKAQSSINSGGSSGGSSGSETPGTSESATPESSGGSSGGSAKNTITKTLQLRIVRPYNSAEVEKIVADEKNNREKVALEKNKDKVKEACSKHLKVASYCTTQVERNACLFCKARKLDDKFYQKLRGQFPDAVFWQEIGEVFRQLQKQAAEIYNQSLIELYYEIFIKGKGFANASSVEHYLSDVCYTRAAELFKNAAIASGLRGKVKSNFRLKELKNMKSGLPTTKSDNFPIPLVKQKGGQYTGFEISSRNDDFIIKIPFGRWQVKKEIDKYRPWEKFDFEQVRKSPKPISLLLSTQRRKRNKGWSKDEGTEAEIRKVMNGDYQTSYIEVKRGSKVGEKSAWMVNLSIDVPKIDKGVDPSIIGGIDVGVKSPLVCAVNNALSRYSIDDNDLFHFNKKMFARRRILLKKSRHKRAGHGAKNKLKPISVLTEKSKRFRKKLIERWAYEIADFFVKNKVGTVQMENLESMKRKEDSYFNIRLRGFWPYAEMQNKIEFKLKQYGIVVRKVAPNNTSKTCSQCGHLNNYFNFEYRKKNKFPYFKCEKCNFKENADYNAALNISNPQLKSTKGEP

SEQ ID NO: 1983 - protein, 726 aa, synthetic construct
SEDEFSHEYWMRHALTLAKRARDGREVPVGAVLVLNNRVIGEGWNRTIGLHDPTAHAEIMALRQGGLVMQNYRLIDATLYVTFEPCVMCAGAMVHSRIGRVVFGVRNSKRGAAGSLMNVLDYPGMGHRVEITEGILADECAALLCDFYCMPRQVFNAQKRAQSSINSGGSSGGSSGSDTPGTSESATPESSGGGSSGSAKNTITKTLQLRIVRPYNSAEVEKIVADEKNNREKIALEKNKDKVREACSKHLKVASYCTTQVERNACPFCKARKLDDKFYQRLRGQFPDAVFWQELGEILRQLQKQAAEIYNQSLIELYYEIFIKGRGFANASSVEHYLSDVCYTRAAELFKNAAIASGLRGKVKGNFRLKELKNMKSGLPTTKSDNFPIPLVKQKGGQYTGFEISNHDGDFIIKIPFGRWQVKKEINKHRPWEKFDFEQVRKSPKPISLLLSTQRRKRNKGWSKDEGTEAEIRKVMNGDYQTSYIEVKRGSKIGEKSAWMLNLSIDVPKIDKGVDPNIIGGIDVGVKSPLVCAINNALSRYSISDNDLFHFNKKMFARRRILLKKSRHKRAGHGTKNKLMPITILTEKSKRFRKKLIERWACEIADFFIKNKVGTVQMENLESMKRKEDSYFNTRLRGFWPYAEMQNKIEFKLKQYGIEIRKVAPNNTSKTCSKCGHLNNYFNFEYRKKNKFPPFKCEKCNFKEDADYNAALNISNPKLKGTKEEP

SEQ ID NO: 1984 - protein, 726 aa, synthetic construct
SEDEFSHEYWMRHALTLAKRARDGREVPVGAVLVLNNRIIGEGWNRAIGLHDPTAHAEIMALRQGGLVLQNYRLIDATLYVTFEPCVMCAGAMVHSRIGRVVFGVRNSKRGAAGSLMNVLDYPGMGHRVEITEGILAEECAALLCDFYCMPRQVFNAQKRAQSSINSGGSSGGSSCSETPGTSESVAPKSSGGSSAGSTKNTITKTLKLRIVRPYNSAEVEKIVADEKNSRERIALEKNKDKVKEACSEHLRVAAYCTTQVERNACLFCKARKLDDKFYQKLRGRFPDAVFWQELGEILRQLQKQAAEIYNQSLIELYYEIFIKGRGFANASSVEHYLSDVCYTRAAELFKNAAIASGLRGKVKSNFRLKELKNMKSGLPTTKSDNFPIPLVKQKGGQYTGFEISSHNDDFIIKIPFGRWQVKKEIDKYRPWEKFDFEQVRKSPKPISLLLSTQRRKRNKGWSKDEGTEAEIRKVMNGDYQTSYIEVKRGSKTGEKSAWMLNLSIDVPKIDKGVDPSIIGGIDVGVKSPLVCAINNAFSRYSISDNDLFRFNKKMFARRRILLKKNRHKRAGHGAKNKLKPISILTGKSERFRKKLIERWACEIADFFTKNKVGTVQMENLESMKRKEDSYFNIRLRGFWPYAEMQNKIEFKLKQYGIEIRKVAPNNTSKTCSKCGHLNNYFNFEYRKKNKFPHFKCEKCNFKENADYNAALNISNPKLKSTKEEP

SEQ ID NO: 1985 - protein, 726 aa, synthetic construct
SEVEFSHEYWMRHALTLAKRARDGREVPVGAVLVLNNRVIGEGWNRAIGLHDPTAHAEIMALRQGGLVMQNYRLIDATLYVTFEPCVMCAGAMIHSRIGRVVFGIRNNKHGAAGSLVNVLNYPGMNHRVEITEGILADECAALLCDFYRMPRQVFNARKKAQSSISPGGSSGGSSGSETPGASESVTPKSSGGSSGGSAKNTITKTLKLRIVRPYNSAKVEKIVADEKNNREKIALEKNKGKVKEACSKHLEVAAYCTTQVERNACLFCKARKLDDKFYQKLRGQFPDAVFWQELGEILRQLQKQAAEIYNQSLIELYYEIFIKGRGFANASSVEHYLSDVCYTRAAELFKNAAIASGLRGKVKGNFRLKELRNMKSGLPTTKSDNFPIPLVKQKGGQYTGFEISSHNDDFIIKIPFGRWQVKKEIDKHRPWEKFNFEQVRKSPKPISLLLSTQRRKRNKGWSKDEGTEAEIRKVMNGDYQTSYIEVKRGSKIGEKSAWMLNLSIDVPKIDKGVDPSIIGGIDVGVKSPLVCAINNAFSRYSISDNDLFHFNKKMFARRRILLKKSKHKRAGHGAKNKLKPITILTEKSERFRKKLIERWACEIADFFIKNKVGTVQMENLESMKRREDSYFNIRLRGFWPYAKMLNRIEFKLKQYGIKIRKVAPNNTSKTCSKCGHLNNYFNFEYRKKNKFPHFKCEKCNFRENADYNAALNISNPKLKSTKGEP

SEQ ID NO: 1986 - protein, 726 aa, synthetic construct
SEVEFSHEYWMRHALTLAKRARDEREVPVGAVLVLNNRVIGEGWNRAIGLHDPTAHAEIMALRQGGLVMQNYRLTDATLYVTFEPCVMCAGAMIHSRIGRVVFGVRNSKRGAAGSLMNVLNYPGMNHSVEITEGILMDECAALLCDFYRMPRQVLNAQKKAQSGFNSGGSSGCGSGSETPGTSESVAPKSSGDSSGGSAKNTITKTLKLRIVRPYNSAEVEKIVADEKNSREKIALEKNKDKVKEACSKHLKVAAYCTTQVERNACLFCKARKLDDKFYQKLRGQFPDAVFWQEIGEIFRQLQKQAAEIYNQSLIELYYEIFIKGKGFANASSVEHYLSDVCYTRAAELFKNAAIASGLRGKVKSNFRLKELKNMKSGLPTTKSDNFPIPLVRQKGGQYTGFEISNHDGDFIIKIPFGRWQVKKEINKHRPWEKFDFEQVRKSPKPISLLLSTQRRKRNKGWSKDEGTEAEIRKVMNGDYQTSYIEVKRGSKIGEKSAWMLNLSIDVPKIDKGVDPSIIGGIDVGVKSPLVCAINNALSRYSISDNDLFHFNKRMFARRRILLRKNRHKRAGHGTKNKLKPITILTEKSGRFRKKLIERWACEIANFFIKNKVGTVQMENLESMKRKEDSYFNIRLRGFWPYAEMQNKIEFKLKQYGIKIRKVAPNNTSKTCSKCGHLNNYFGFEYRRKNKFPHFKCEKCNFKEDADYNAALNISNPKLKSTKEEP

SEQ ID NO: 1987 - protein, 726 aa, synthetic construct; identical to SEQ ID NO: 684

SEQ ID NO: 1988 - protein, 726 aa, synthetic construct
SEVEFSHEYWMRHALTLAKRARDEREVPVGAVLVLNNRVIGVGWNRAVGLHDPTAHAEIMALRQGGLVMQKYRLIEATLYVTFEPCIMCAGAMIHSRIGRVVFGVRNSKRGAAGSLMNVLDYPGMNHRVGITEGILADECAALLCDYYRMPRQVFNARKKAQSSINSGGSSDGGSGSETPGTSESATPKSSGGSSGGSAKNTITKALKLRIVRPYNSAEVEKIVADEKNNREKIALEKNKDKVKEACSEHLKVAAYCTTQVERNACLFCKARKLDDKFYQKLRGQFPDAVFWQELGEIFRQLQKQTAEIYNQSLIELYYEILIKGKGFANASSVEHYLSDVCYTRAAELFKNAAIASGLRGKVKSNFRLKELKNMRSGLPTTKSDNFPIPLVKQKGGQYTGFEISSHNDDFIIKIPFGRWQVKKEIDKYRPWERFDFEQVRKSPKPISLLLSTQRRKRNKGWSKDEGTEAEIRKVMNGDYQTSYIEVKRGSKIGEKSAWMLNLSIDVPKIDKGVDPSIIGGIDVGVKSPLVCAINNAFSRYSISDNDLFRFNKKMFARRRILLKKNRHKRAGHGAKNKLKPISILTGKSERFRKKLIERWACEIADFFIKNKVGTVQMENLEGMKRKEDSYFNIRLRGFWPYAEMQNKIEFKLKQYGIEIRKVAPNNTSKTCSKCGHLNNYFNFEYRKKNKFPHFKCEKCNFKENADYNAALNISNPKLKSTKEEP

SEQ ID NO: 1989 - protein, 726 aa, synthetic construct
SEVEFSHEYWMRHALTLAKRARDEREVPVGAILVLNNRVIGEGWNRAIGLHDPTAHAEIMALRQGGLVMQNYRLIDATLYVTFEPCVMCAGAMIHSRIGRVVFGVRNSKHGAAGSLVNVLNYPGMNHRVEITEGILADECAALLCDFYRMPRQVLNARKKAQSSINPSGSSGGSSGSETPGTSESPTPESSGGSPGGSAKNTITKTLKLRIVRPYNSTEVEKIVADEKNNREKIALEKNKDKVKEACSKHLKVAAYCTTQVERNACLFCKARKLDDKFYQKLRGQFPDAVFWQEIGEIFRQLQKQAAEIYNQSLIELYYEIFIKGKGFANASSVEHYLSDVCYSRAAELFKNAAIASGLRGKVKSNFRLKELKNMKSGLPTTKSDNFPIPLVKQKGGQYTGFEISSHNDDFIIKIPFGRWQVKEEIDKYRPWEKFGFEQVRKNPKPISLLLSTQRRKRNKGWSKDEGTEAEIRKVMNGDYQTSYIEVKRGSKIGEKSAWMLNLSIDVPKIDKGVDPSIIGGIDVGVKSPLVCAINNALSRYSISDNDLFHFNKKMFARRRILLRKNRHKRAGHGAKNKLKPITIMTEKSKRFRKKLIERWACEIADFFIKNKVGTVQMENLESMKRKEDSYFNIRLRGFWPYAEMQNKIEFKLKQYGIVVRKVAPNNTSKTCSKCGHLNNYFNFEYRKKNKFPHFKCKKCNFKESADYNAALNISNPKLKSTKEEP

SEQ ID NO: 1990 - protein, 726 aa, synthetic construct
SEVEFSHEYWMRHALTLAKRARDEREVPVGAILVLNNRVIGEGWNRAIGLHDPTAHAEIMALRQGGLVMQNYRLTEATLYVTFEPCVMCAGAMIHSRIGRVVFGVRNSKRGAAGSLMNVLNYPGMNHCVEITEGILVDECAALLCDFYRMPRQVLNAQKKAQSSISSGGSSGGSSGSETPGASESATPGGSGGSSGGSAKNTITKTLKLRIVRPYNSAEVEKIVADEKNNREKIALEKNKDKVKEACSKHLKVASYCTTQVERNACLFCKARKLDDKFYQKLRGQFPDAVFWQEISEIFRQLQKQAAEIYNQSLIELYYEIFIKGRGFANASSVEHYLSDVCYTRAAELFKNAAIASGLRGKVKSNFRLKELKSMKSGLPTTKSDNFPIPLVKQKGGQYTGFEISSHNDDFIIKIPFGRWQVKKEIDKYRPWEKFDFEQVRKNPKPISLLLSTQRRKRNKGWSKDEGTEAEIRKVMNGDYQTSYIEVKRGSKIGEKSAWMLNLSIDVPKIDKGVDPSIIGGIDVGVKSPLVCAINNAFSRYSISDNDLFHFNKKVFARRRILLKKNRHKRAGHGTKNKLKPITILTEKSGRFRKKLIERWACEIADFFIKNKVGTVQMENLESMKRKEDSYFNIRLRGFWPYAEMQNKIEFKLKQYGIEIRRVAPNNTSRTCSKCGHLNNYFNFEYRRKYKFPHFKCEKCNFKEDADYNAALNISNPKLKSTKEEP

SEQ ID NO: 1991 - protein, 726 aa, synthetic construct
SEDEFSHEYWMRHALTLAKRARDGREVPVGAVLVLNNRVIGEGWNRAIGLHDPTAHAEIMALRQGGLVMQNYRLIDATLYVTFEPCVMCAGAMVHSRIGRVVFGVRNSKRGAAGSLMNVLNYPGMGHRVEITEGILADECAALLCDFYCMPRQVFNAQKRAQSNINSGGSSGGSSGSETPGSSESATPESSGGGSSGSAKNTITKTLQLRIVRPYNSAEVEKIVADEKNNREKIALEKNKDKVKEACSKHLKVASYCTTQVERNACPFCKARKLDDKFYQKLRGQFPDAVFWQELGEILRQLQKQAAEIYNQSLIELYYEIFIKGRGFANAGSVEHYLSDVCYTRAAELFKNAAIASGLRGKVKSNFRLKELKNMKSGLPTTKSDNFPIPLVKQKGGQYTGFEISSHNDDFIIKIPFGRWQVKKEVDRYRPWEKFDFEQVRKSPKPISLLLSTQRRKRNRGWSKDEGTEAEIKKVMDGDYQTSYIEVKRGSKIGEKSAWMLSLSIDVPKIDKGVDPSIIGGIDVGVKSPLVCAINNAFSRYSISDNDLFHFNKKVFARRRILLKKNRHRRAGHGAKNKLKPITILTEKSKRFRKKLIERWACEIADFFVKNKVGTVQMENLESMKRKEDSYFNIRLRGFWPYAEMQNKIEFKLKQYGIEIRKVAPNNTSKTCSKCGHLNNYFNFEYRKKNKFPHFKCEKCNFKEDADYNAALNISNPKLRSTKEEP

SEQ ID NO: 1992 - protein, 726 aa, synthetic construct
SEVEFSHEYWMRHALTLAKRAHDEREVPVGAILVLNNRVIGEGWNRAIGLHDPTAHAEIMALRQGGLVMQNYRQIDATLYVTFEPCVMCAGAMIHSRIGRVVFGVRNSKHGAAGSLMNVLNYPGMNHRVEITEGILADECAALLCDFYRMPHQVFNARKKAQSSINPGGPSGGSSGSETPDTSESATPESSGGSSGSSAKNTITKTLKLRIVRPYNSAEVEKIVADEKNNREKIALEKNKDKVKEACSKHLKVASYCTTQVERNACLFCKARKLDDKFYQKLRGQFPDAVFWQEIGEIFRQLQKQAAEIYNQSLIELYYEIFIKGRGFANASSVEHYLSDVCYTRAAELFKNAAIASGLRGKVKSNFRLKELKNMKSGLPTTKSDNFPIPLVKQKGGQYTGFEISSHNDDFIIKIPFGRWQVKKEIDKYRPWEKFDFEQVRKSPKPISLLLSTQRRKRNKGWGKDGGTEAEIRKVMNGDYQTSYIEVKRGSKTGEKSAWMLNLSIDVPKIDKGVDPSIIGGIDVGVKSPLVCAINNAFSRYSISDNDLFRFNKKMFARRRILLKKNRHKRAGHGVKNKLKPISILTGKSERFRKKLIERWACEIADFFIKNKVGTVQMENLESMKRKEDSYFNIRLRGFWPYAEMQNKIEFKLKQYGIEIRKVAPNNTSKTCSKCGHLNNYFNFEYRKKNKFPHFKCEKCNFKENADYNAALNISNPKLKSTKGEP

SEQ ID NO: 1993 - protein, 726 aa, synthetic construct
SEVEFSHEYWMRHALTLAKRARDEREVPVGAVLVLNNRVIGEGWNRAIGLHDPTAHAEIMALRQGGLVMQNYRLVNATLYVTFEPCVMCAGAMIHSRIGRVVFGVRNSKRGAAGSLMNVLNYPGMNHRVEITEGILADECAAPLCDFYRMPRQVFNAQKKAQSSTNSGGSSGGSSGSETLGTREGATPESSGGSSGGSAKNTITKTLKLRIVRPYNSAEVEKIVVDEKNNREKVALEKNKDKVKEACSEHLKVAAYCTTQVERSACLFCKARKLDDKFYQKLRGQFPDAVFWQEIGEVFRQLQKQAAEIYNQSLIELYYEIFIKGKGFANASSVEHYLSDVCYTRAAELFKNAAIASGLRGKVKSNFRLKELKNMKSGLPTTKSDNFPIPLVKQKGGQYTGFEISSHNDDFIIKIPFGRWQVKKEINKFRPWEKFDFEQVRKSPKPISLLLSTRRRKRNKGWSKDEGTEAEIRKVMNGDYQTSYIEVKRGSKIGEKSAWMLNLSIDVPKIDKGVDPGIIGGIDVGVRSPLVCAINNAFSRYSISDNDLFRFNKKMFARRRILLKKNRHKRAGHGAKNKLKPISILTGKSERFRKKLIERWACEIADFFIKNKVGTVQMENLESMKRKEDSYFNIRLRGFWPYAEMQNKIEFKLKQYGIEIRKVAPNNTSKTCSKCGHLNNYFNFEYRKKNKFPHFKCEKCNFKENADYNAALNISNPKLKSTKEEP

SEQ ID NO: 1994 - protein, 726 aa, synthetic construct; identical to SEQ ID NO: 1986

SEQ ID NO: 1995 - protein, 726 aa, synthetic construct
SEVEFSHEYWMRHALTLAKRARDEREVPVGAVLVLNNRVIGEGWNRAIGLHDPTAHAEIMALRQGGLVMQNYRLTDATLYVTFEPCVMCAGAIIHSRIGRVVFGVRNSKRGAAGSLMNVLNHPGMNHRVEITGGILADECAALLCDFYRMPRQVFNAQKKARSNINSGGSSGGSSGSETLGTSESATPESSGGSSGGSAKNTITKTLKLRIVRPYNSAEVEKIVADEKNNREKIALEKNKDKVKEACSEHLKVAAYCTTQVERNACLFCKARKLDDKFYQKLRGQFPDAVFWQEIGEIFRQLQRQAAEIYNQSLIELYYEIFIKGKGFANASSVEHYLSDVCYARAAELFKNAAIASGLRGKVKSNFRLKELKNMKSGLPTTKSDNFPIPLVKQKGGQYTGFEISSHNDDFIIKIPFGRWRVKKEIDKYRPWEKFDFEQVRKSPKPISLLLSTQRRKRSKGWSKDEGTEAEIRKVMNGDYQTSYIEVKRGSKIGEKSAWMLSLSIDVPKIDKGVDPSIIGGIDVGVKSPLVCAINNAFCRYSISDNDLFHFNKKMFARRRILLKKSRHKRAGHGAKNKLKPISILTEKSKRFRKKLIERWACEIADFFIKNKVGTVQMENLESMKRKEDSYFNIRLRGFWPYAEMQNKIEFKLKQYGIEIRKVAPNNTSKTCSKCGHLNNYFNFEYRKKNKFPHFKCEKCNFKENADYNAALNISNPKLKSAKEEP

SEQ ID NO: 1996 - protein, 726 aa, synthetic construct
SEDEFSHEYWMRHALTLAKRARDGREVPVGAVLVLNNRVIGEGWNRAIGLHDPTAHAEIMALRQGGQVMQNYRLIDATLYVTFEPCVMCAGAMVHSRIGRVVFGVRNSKRGAAGSLMNVLDYPGMGHRVEITEGILADECAALLCDFYCMPRQVFNAQKRAQSSINSGGSSGGSSGSDTPGTSESATPESSGGGSSGSAKNTITKTLQLRIVRPYNSAEVEKIVADEKNNREKIALEKNKDKVREACSKHLKVASYCTTQVERNACLFCKARKLDDKFYQKLRGQFPDAVFWQELGEILRQLQKQAAEIYNQSLIELYYEIFIRGRGFANASSVEHYLSDVCYTRAAELFKNAAIASGLRNKIKSNFRLKELRNMKSGLPTTKSDNFPIPLVRQKGGQYTGFEISNHDGDFIIKIPFGRWQVKKEINKHRPWEKFDFEQVRKSPKPISLLLSTQRRKRNKGWSKDEGTEAEIRKVMNGDYQTSYIEVKRGSKIGEKSAWMLNLSIDVPKIDKGVDPSIIGGIDVGVKSPLVCAINNALSRYSISDNDLFHFNKKMFARRRILLRKNRHKRAGHGAKNKLKPITIMTEKSKRFRKKLIERWACEIADFFIKNKVGTVQMENLESMKRKEDSYFNIRLRGFWPYAEMQNKIEFKLKQYGIVVRKVAPNNTSKTCSKCGHLNNYFNFEYRKKNKFPHFKCEKCNFKEDADYNAALNISNPKLKSTKGEP

SEQ ID NO: 1997 - protein, 726 aa, synthetic construct
SEVEFSHEYWMRHALTLAKRARDEREVPVGAVLVLNNRVIGEGWNRAIGLHDPTAHAEIMALRQGGLVMQNYRLTDATLYVTFEPCVMCAGAMIHSRIGRVVFGVRNSKRGAAGSLMNVLNYPGMNHCVEITEGILVDECAALLCDFYRMPRQVLNAQKKAQSSISSGGSSGGSSGSETPGASGSVTPKSSGGSSAGSTKDTITKTLQLRIVRPYNSAEVEKIVADEKNNREKIALEKNKDKVKEACSKHLKVASYCTTQVERNACLFCKARKLDDKFYQKLRGQFPDAVFWQELGEIFRQLQKQAAEIYNQSLIELYYEIFIKGKGITNASRVEHYLSDVCYTRAAELFKNAAIASGLRNKVKSNFRLKELRNMKSGLPTTKSDNFPIPLVRQKGGQYTGFEISNHNGDFIIKIPFGRWQVKKEINKHRPWEKFDFEQVRKSPKPISLLLSTQRRKGNKGWSKDEGTEAEIRRVMNGDYQTSYIEVKRGSKIGEKSAWMLNLSIDVPKIDKGVDPSIIGGIDVGVKSPLVCAINNALSRYSISDNDLFHFNKKMFARRRILLRKNRHKRAGHGARNKLKPITVLTEKCERFRKKLIERWAREIANFFVKNKVGTVQMENLESMKRREDSYFNIRLRGFWPYAEMQNKIEFKLKQYGIEIRKVAPNNTSRTCSKCGHLNNYFNFEYRKKNKFPHFKCEKCNFKENADYNAALNISNPKLKSTKGEP

SEQ ID NO: 1998 - protein, 726 aa, synthetic construct
SEVEFSHEYWMRHALTLAKRARDEREVPVGAVLVLNNRVIGEGWNRTTGLHDPTAHAEIMALRQGGLVMRNYRLTDATLYVTFEPCVMCAGAMIHSRIGRVVFGVRNSKRGAAGSLMNVLNYPGMNHCVEITEGILVDECAALLCDFYRMPRQVLNAQKKALSSISPGGSSGGSSGSETPGASESVTPKSSGGSSGGSAKNTITKTLKLRIVRPYNSAEVEKIVADEKNNREKIALEKNKGKVKEACSKHLEVAAYCTTQVERNACLFCKARKLDDKFYQKLRGQFPDAVFWQELGEIFRQLQKQAAEIYNQSLIELYYEIFIKGKGITNASRVEHYLSDVCYTRAAELFKNAAIASGLRSKVRSNFRLKELKNMKSGLPTTKSDNFPIPLVKQKGGQYTGFEISSHNDDFIIKIPFGRWQVKEEVDKYRPWEKFDFEQVRKSPKPISLLLSTQRRKRNKGWSKDEGTEAEIRKVMNGDYQTSYIEVKRGSKIGEKSAWMLNLSIDVPKIDKGVDPSIIGGIDIGVKSPLVCAINNAFSRYSISDNDLFHFNKRMFARRRILLKKNRHRRAGHGAKNKLKPITVLTEKSERFRKKLIERWACEIADFFIKNKVGTVQMENLESMKRKEDSYFNIRLRGFWPYAEMQNKVEFKLKQYGIVVRKVAPNNTSKTCSKCGHLNNYFNFEYRKKNKFPHFKCERCSFKENADYNAALNISNPKLKSTKEEP

SEQ ID NO: 1999 - protein, 726 aa, synthetic construct
SEVEFSHEYWMRRALTLAKRARDEREVPVGAVLVLNSRVIGVGWNRAISLHDPTAHAEIMALRQGGLVMQNHRLIDATLYVTFEPCVMCAGAMVHSRIGRVVFGVRNSRRGAAGSLMNVLNYPGMNHRVEITEGILADECAALLCDFYRMPRRVFNAQKKAQSNINPGGSSGGSGGSETPGTSESATPKSSGGSSGGSAKNTITKTLKLRIVRPYNSAEVEKIVADEKNNREKIALEKNKDKVKEACSKHLKVAAYCTTQVERNACLFCKARRLDDKFYQKLRGQFPDAVFWQEIGEIFRQLQKQAAEIYNQSLIELYYEIFIKGKGFANASSVEHYLSDVCYTRAAELFKNAAIASGLRGKVKSNFRLKELKSMKSGLPTTKSDNFPIPLVKQKGGQYTGFEISSHNDDFIIKIPFGRWQVKKEIDKYRPWEKFDFEQVRKSPKPISLLLSTRRRKRNKGWSKDEGTEAEIRKVMNGDYQTSYIEVKRGSKIGEKSAWMLNLSIDVPKIDKGVDPSIIGGIDVGVKSPLVCAINNAFSRYSISDNELFHFNKKMFARRRILLRKNRHKRAGHGAKNKLKPITILTEKSERFRKKLIEKWACEIADFFIKNKVGTVQMENLENMKRREDSYFNIRLRGFWPYAEMQNKIEFKLKQYGIEIRRVAPNNTSKTCSKCGHLNNHFNFEYRKKNKFPHFKCEKCNFKESADYNAALNISNPKLKSTKEEP

SEQ ID NO: 2000 - protein, 726 aa, synthetic construct
SEVEFSHEYWMRHALTLAKRARDEREVPVGAILVLNNRVIGEGWNRAIGLHDPTAHAEIMALRQGGLVTQNYRLIDATLYVTFEPCVMCAGAMIHSRIGRVVFGVRNSKHGAAGSLVNVLNYPGMNHRVEITEGILADECAALLCDFYRMPRQVFNAQKKAQSSISSGGSSGGSGGGETPGASESVTPKSSGGSSAGSTKNTITKTLKLRIVRPYNSAEVEKIVADEKNSREKIALEKNKGKVKEACSEHLKVAAYCTTQVERSACPFCKARKLDDRFYQKLRGQFPDAVFWQEISEIFRQLQKQAAEIYNQSLIELYYEILIKGKGFANASSVEHYLSDVCYTRAAELFKNAAIASGLRGKVKSNFRLKELKNMKSGLPTTKSDNFPIPLVKQKGGQYTGFEISSRNDDFIIKIPFGRWQVKKEIDKYRPWEKFDFEQVRKSPKPISLLLSTQRRKRNRGWGKDEGTEAEIKRVMNGDYQTSYIEVKRGSKIGEKSAWMLNLSIDVPKIDKGVDPSIIGGIDVGVKSPLVCAINNAFSRYSISDNDLFRFNKKMFARRRILLRKNRHKRAGHGAKNKLKPISILTGKSERFRKKLIERWACEIADFFIKNKVGTVQMENLESMKRKEDSYFNIRLRGFWPYAEMQNKIEFKLKQYGIEIRKVAPNNTSKTCSKCGHLNNYFNFEYRKKNKFPHFKCEKCNFKENADYNAALNISNPKLKSTKEEP

SEQ ID NO: 2001 - protein, 726 aa, synthetic construct
NEDEFSHEYWMRHALTLAKRARDGREVPVGAVLVLNNRVIGEGWNRAIGLHDPTAHAEIMALRQGGLVMQNYRLIDATLYVTFEPCVMCAGAMVHSRIGRVVFGVRNSKRGAAGSLMNVLDYPGMGHRVEITEGILADECAALLCDFYCMPRQVFNAQKRAQSSINSGGSSGGSSGSETPGTSESATPESSGGGSSGSAKNTITKTLQLRIVRPYNSAEVEKIVADEKNNREKIALEKNKDKVKEACSKHLKVASYCTTQVERNACPFCKARKLDDKFYQKLRGQFPDAVFWQELGEILRQLQKQAAEIYNQSLIELYYEIFIKGRGFANASSVEHYLSDVCYTRAAELFKNAAIASGLRGKVKSNFRLKELRNMRSGLPTTKSDNFPIPLVRQKGGQYTGFEISNHNSDFIIKIPFGRWQAKKEIDKYRPWEKFDFEQVRKSPKPISLLLSTQRRKRNKGWSKDEGTEAEIRRVMNGDYQTSYIEVKRGSKIGEKSAWMLSLSIDVPKIDKGVDPRIIGGIDVGVKSPLVCAINNVLSRYSISDNDLFHFNKKMFARRRILLKKNGHKRAGHGAENKLKPITIMTEKSKRFRKKLIERWACEIADFFIKNKVGTVQMENLESMKRKEDSYFNIRLRGFWPYAEMQNKIEFKLKQYGIVVRKVAPNNTSKTCSQCGHLNNYFNFEYRKKNQFPYFKCEKCNFKENADYNAALNISNPQLKSTKGEP

SEQ ID NO: 2002 - protein, 726 aa, synthetic construct
SEVEFSHEYWMRHALTLAKRARDEREVPVGAVLVLNNRVIGVGWNRAIGLHDPTAHAEIMALRQGGLVMQNYRLIDATLYVTFEPCVMCAGAMIHSRIGRVVFGVRNNKHGAAGSLVNVLNYPGMNHRVEITEGILADECAALLCDFYRMPRQVFNARKKAQSSINPSGSSGGSSGSETPGTSESATPESSGGSSGGSAKNTITKTLKLRIVRPYNSAEVEKIVADEKNSREKIALEKNKDKVKEACSEHLKVAAYCTTQVERNACLFCKARKLDDRFYQKLRGQFPDAVFWQEIGEIFRQLQKQAAEIYNQSLIELYYEIFIKGKGFANASSVEHYLSDVCYTRAAELFKNAAIASGLRGKVKSNFRLKELKNMKSGLPTTKSDNFPIPLVKQKGGQYTGFEISSHNDDLIVKIPFGRWQVKKEIDRYRPWEKFDFEQVRKSPKPISLLLSTQRRKRNKGWSKDEGTEAEIRKVMNGDYQTSYIEVKRGSRIGEKSAWMLSLSIDVPKIDRGVDPSIIGGIDVGVKSPLVCAISNALSRYSISDNDLFHFNKKMFARRRILLKKNRHRRAGHGARNKLKPITVLTEKSKRFRKKLIERWACEIANFFIKNKVGTVQMENLESMKRKEDSYFNIRLRGLWPYAEMQNKIEFKLKQYGIEIRKVAPNNTSKTCSKCGHLNNYFNFEYRKRNKFPHFKCEKCNFKENADYNAALNISNPKLKSTKGEP

SEQ ID NO: 2003 - protein, 726 aa, synthetic construct
SEVEFSHEYWMRHALTLAKRARDEREVPVGAILVLNNRVIGEGWNRAIGLHDPTAHAEIMALRQGGLVMQNYRLIDATLYVTFEPCVMCAGAMIHSRIGRVVFGVRNSKHGAAGSLVNVLNHPGMNHRVEITEGILADECAALLCDFYRMPRQVFNARKKAQSSINPGGSSGGSSGSETPGTSESATPESSGGGSSGSAKNTITKTLQLRIVRPYNSAEVEKIVADEKYNREKIALEKNRDKVKEACSEHLKVAAYCTTRVERNACLFCKARKLDDRFYQKLRGQFPDAVFWQEIGEIFRQLQKQAAEVYNQSLIELYYEIFIKGKGFANASSVEHYLSDVCYARAAELFKNAAIASGLRGKVKSNFRLKELKNMKSGLPTTKSDNFPIPLVKQKGGQYTGFEISSRNDDFIIKIPFGRWQGKKEVDKYRPWEKFDFEQVRKSPKPISLLLSTQRRKRNKGWSKDEGTEAEIKKVMNGDYQTSYIEVKRGSKIGEKSAWMLSLSIDVPKIDRGVDPSIIGGIDVGVKSPLVCAINNASSRLSISDNDLFRFNKKMFARRRILLKKNGHKRAGHGAKNKLKPITILTEKSVRFRKKLIERWACEIADFFIRNKVGTVQMENLESMKRKEDSYFNIRLRGFWPYAEMQNKIEFKLKQYGIEIRKVAPNNTSKTCSKCGHLNNYFNFEYRKKNKFPHFKCEKCNFKENADYNAALNISNPKLRSTKEEP

SEQ ID NO: 2004 - protein, 726 aa, synthetic construct
SEVEFSHEYWMRHALTLARRARGEREVPVGAILVLNNRVIGEGWNRAIGLHDPTAHAEIMALRQGGLVMQSYRLADATLYVTFEPCVMCAGAMIHSRIGRVVYGVRNSKHGAAGSLMNVLNYPGMNHRVEITEGILADECAALLCDFYRMPRRVFNAQKKAQSSINSGGSSDGSSGSGTLGTSRSPTRESSGGSSGGSAKNTITKTLKLRIVRPYNSAEVEKIVADEKNNREKIALEKNRGKVKEACSKHLKVAAYCTTQVERNACLFCKARKLDDKFYQKLRGQFPDAVFWQEIGEIFRQLQKQAAEIYNQSLIELYYEVFIKGRGFANASSVEHYLSDVCYTRAAELFKNAAIASGLRGKVKGNFRLKELKNMKSGLPTTKSDNFPIPLVKQKGGQYTGFEISSHNDDFIIKIPFGRWQVKKEIDKYRPWEKFDFEQVRKSPKPISLLLSTQRRKRNKGWSKDEGTEAEIRKVMNGDYQTSYIEVKRGSKIGEKSAWMLNLSIDVPKIDKGVDPSIIGGIDVGVKSPLVCAINNAFSRYSIGDNDLFHYNKKMFARRRILLKKNRHKRAGHGAKNKLKPISILTEKSKRFRRKLIERWACEIADFFIKNKVGTVQIENLESMKRKEDSYFNIRLRGFWPYAEMQNKIEFKLKQYGIEIRKVAPNNTSKTCSKCGHLNSYFNFEYRKKNKFPHFKCEKCNFKENADYNAALNISNPKLKSTKEEP

SEQ ID NO: 2005 - protein, 726 aa, synthetic construct
SEVEFSHEYWMRRALTLAKRARDEREVPVGAVLVLNNRVIGEGWNRTTGLHDPTAHAEIMALRQGGLAMQNYRLTGATLYVTFEPCVMCAGAMIHSRIGRVVFGVRNSKRGAAGSLTNVLNYPGMNHRVEITEGILVDECAALLCDFYRMPRQVFNAQKKAQSTINSGGSSGGSSGSETPGTSESPTPESSGGSPGGSAKNTITKTLKLRIVRPYNSAEVEKIVADEKNNREKIALEENKDKVKEACSKHLKVAAYCTTQVERNACLFCKARKLDDKFYQKLRGQFPDAVFWQEIGEIFRQLQKQAAEIYNQSLIELYYEIFIKGRGFANASSVEHYLSDVCYTRAAELFKNAAIASGLRGKVKSNFRLKELKSMKSGLPTTKSDNFPIPLVKQKGGQYTGFEISSHNDDFIIKIPFGRWQEKKEINKYRPWERFDFEQVRKSPKPISLLLSTQRRKRNKGWGKDEGTEAEIKKVMNGDYQTSYIEVKRGSKIGEKGAWMLNLSIDVPKIDKGVDPSIIGGIDVGVKSPLVCAINNAFSRYSISDNDLFRFNKKMFARRRILLKKNRHKRAGHGARNKLKPITILTEKSERFRKKLIERWASEIADFFIKNKVGTVQMENLESMKRKEDSYFNIRLRGFWPYAEMQNKIEFKLKQYGIEIRKVAPNNTSKTCSKCGHLNNYFNFEYRKKNKFPHFKCEKCNFKEDADYNAALNISNPKLKSTKEEP

SEQ ID NO: 2006 - protein, 726 aa, synthetic construct
SEVEFSHEYWMRHALTLAKRARDEREVPVGAILVLNNRVIGEGWNRAIGLHDPTAHAEIMALRQGGLVMQNYRLIDATLYVTFEPCVMCAGAMIHSRIGRVVFGVRNNKHGAAGSLVNVLNYPGMNHRVEITEGILANECAALLCDFYRMPRQVFNARKKAQSSINPSGSSGGSSGSVTPGTSESATPESSGGGSGGSAKNTITKTLQLRIVRPYNSAEVEKIVTDEKNNREKIALEKNKDKVKEACSKHLKMASYCTTQVERNACLFCKARKLDDKFYQKLRGQFPDAVFWQELGGIFRQLQKQAAEIYNQSLIELYYEIFIKGKGITNASRVEHYLSDVCYTRAAELFKNAAIASGLRSKVRSNFRLKELKNMKSGLPTTKSDNFPIPLVKQKGGQYTGFEISSHNDDFVIKIPFGRWQVKKEIDKYRPWEKFDFEQVRKSPKPISLLLSTQGRKRNKGWSKDEGTEAEIRKVMNGDYQTSYIEVKRGSKIGEKSAWVLNLSIDVPKIDKGVDPSIIGGIDVGVRSPLVCAINNAFSRYSISDNDLFRFNKKMFARRRILLKKNRHKRAGHGAKNKLKPITVLTEKSERVRKKLIERWACEIANFFIKNKVGTVQMENLESMKRREDSYFNIRLRGFWPYAEMQSKIEFKLKQYGIEVRKVAPNNTSKTCSKCGHLNNYFNFEYRKKNKFPHFKCEKCNFKEDADYNAALNISNPKLKGTKEEL

SEQ ID NO: 2007 - protein, 726 aa, synthetic construct
SEVEFSHEYWMRHALTLAKRARDEREVPVGAVLVLNNRAIGEGWNRAIGLHDPTAHAEIMALRQGGLVMQNYRLTDATLYVTFEPCVMCAGAMIHSRIGRVVFGVRNSKRGAAGSLMNVLNYPGMNHCVEITEGILVDECAALLCDFYRMPRQVLNTQKKAQSSISPGGSSGGSSGSETPGASESVTPESSGGSSGSSAKNTITKTLKLRIVRPYNSAEVEKIVADEKNNREKIALEKNKDKVKEACSKHLKVAAYCTTQVGRNACLFCKARRLDDKFYQKLRGQFPDAVFWQEIGEIFRQLQKQAAEVYNQSLVELYYEILIKGKGIANASSVEHYLSDVCYTRAAELFKNAAIASGLRNKIKSNFRLKELRNMKSGLPTTKSDNFPIPLVRQKGGQYTGFEISSHNDDFIIKIPFGRWQVKKEIDKYRPWEKFDFEQVRKSPKPISLLLSTQRRKMNKGWSKDEGTEAEIRKVMNGDYQTSYIEVKRGSKIGEKSAWMLNLSIDVPKIDKGVDPSIIGGIDVGVKSPLVCAINNSSSRYSICDNDLFRFNKKMFARRRILLKKNRHRRAGHGARNKLKPITVLTEKSKRFRKKLIERWACEIANFFIKNKVGTVQMENLESMKRKEDSYFNIRLRGLWPYAEMQNKIEFKLKQYGIEIRKVAPNNTSKTCSKCGHLNNYFNFEYRKRNKFPHFKCEKCNFKENADYNAALNISNPKLKGTKEEP

SEQ ID NO: 2008 - protein, 726 aa, synthetic construct
SEVEFSHEYWMRHALTLAKRARDEREVPVGAVLVLNNRVIGEGWNRAIGLHDPTAHAEIMALRQGGLVMQNYRLVDATLYVTFEPCVLCAGAMVHSRIGRVVFGVRNSKRGAAGSLMNVLNYPGMNHRVEITEGILADECAALLCDFYRMPRQVFNARKRARSNINSGGSSGGSSGSETVGTREGATPESSGGSSGGSAKNTITKTLKLRIVRPYNSAEVEKIVVDEKNNREKVALEKNKDKVKEACSEHLKVAAYCTTQVERSACLFCKARKLDDKFYQKLRGQFPDAVFWQEIGEIFRQLQKQAAEIYNQSLIELYYEIFIKGKGFANASSVEHYLSDVCYTRAAELFKNAAIASGLRGKVKSNFRLKELKNMRSGLPTTKSDNFPIPLVKQKGGQYTGFEISSHNDDFIIKIPFGRWQVKKEIDKYRPWEKFDFEQVRKSPKPISLLLSTQRRKRNKGWSKDEGTEAEIRKVMNGDYQTSYIEVKRGSKIGEKSAWMLNLSIGVPKIDKGVDPSIIGGIDVGVKSPLVCAINNAFSRYSISDNDLFHFNKKMFARRRILLKKNRHKRAGHGAKNKLKPISILTEKSKRFRKKLIERWACEIADFFIKNKVGTVQMENLESMKRKEDGYFNIRLRGFWPYAEMQNKIEFKLKQYGIEIRKVAPNNTSKTCSKCGHLNNYFNFEYRKTNKFPHFKCEKCNFKEDADYNAALNISNPKLKSTKEEP

SEQ ID NO: 2009 - protein, 726 aa, synthetic construct
SEVEFSHEYWMRRALTLAKRARDEREVPVGAVLVLNNRVIGEGWNRAIGLYDPTAHAEIMALRQGGLVMQNYRLVDATLYVTFEPCVMCAGAMVHSRIGRVVFGVRNSKRGAAGSLMNVLDYPGMGHRVEITEGILADECAALLCDFYCMPRQVFNARKKAQSSINPGGPSGGSSGSGMPDTSESATPESSGGNSGGSAKNTITKTLKLRIVRPYNSAEVEKIVADEKNNREKIALEKNKDKVKEACSKHLKVAAYCTTQVERNACLFCKARKLDDKFYQKLRGQFPDAVFWQEIGEIFRQLQKQAAEIYNQSLIELYYEIFIKGKGFANASSVEHYLSDVCYTRAAELFKNAAIASGLRGKVKSNFRLKELKNMKSGLPTTKSDNFPIPLVRQKGGQYTGFEISSHNDDFIIKIPFGRWQVRKEIDKYRPWEKFDFEQVRKSPKPISLLLSTQRRKRNKGWSKDEGTEAEIRKVMNGDYQTSYIEVKRGSKTGEKNAWMLNLSIDVPKIDKGVDPSVIGGIDVGVKSPLVCAINNAFSRFSISDNDLFHFNKKMFARRRILLKKNGRKRAGHGAKNKLRPITILTEKSKRFRKKLIERWACEIAGFFIKNKVGTVQMENLESMKRKEDSYFNIRLRGFWPYAEMQNKIEFKLKQYGIKIRKVAPNNTSRTCSRCGHLNNYFSFEYRKKNKFPHFKCEKCNFKENADYNAALNISNPKLKSTKEEP

SEQ ID NO: 2010 - protein, 726 aa, synthetic construct
SEVEFSHEYWMRHALTLAKRARDEREVPVGAVLVLNNRVIGVGWNRAIGLHDPTAHAEIMALRQGGLVTQNYRLIDATLYVTFEPCIMCAGAMIHSRIGRVVFGVRNSKRGAAGSLMNVLDYPGMNHRVEITEGILAGECAALLCDFYRMPRQVFNAQKKAQSNINPGGSSEGSSGSETPGTSESPTPESSGGSSGGSAKNTITKTLKLRIVRPYNSAEVEKIVADEKNNREKIALEKNKDKVKEACSEHLKVAAYCTTQVERNACLFCKARKLDDRFYQKLRGQFPDAVFWQEIGEIFRQLQKQAAEIYNQSLIELYYEIFIKGKGFANASSVEHYLSDVCYTRAAELFKNAAIASGLRGKVKSNFRLKELKNMKSGLPTTKSDNFPIPLVKQKGGKYTGFEISSHNDDFIIKIPFGRWQVKKEIDKYRPWEKFDFEQVRKSPKPISLLLSTQRRKRNKGWSKDEGTEAEIRKVMNGDYQTSYIEVKRGSKIGEKSAWMLSLSIDVPKIDKGVDPSIIGGIDVGVKSPLVCAINNALSRYSISDNDLFHFNKKMFARRRILLKKNRHKRAGHGAKNKLKPFTVLTEKSERFRKKLIERWACEIANFFIKNKVGTVQMENLESMKGKEDSYFNIRLRGFWPYAEMQNKIEFKLKQYGIEIRKVAPNNTSKTCSKCGHLNNYFNFEYRRKNKFPHFKCEKCNFKENADYNAALNISNPKLKGTKEEP

SEQ ID NO: 2011 - protein, 726 aa, synthetic construct
SEVEFSHEYWMRHALTLAKRARDEREVPVGAVLVLNNRVIGVGWNRGIGLHDPTAHAEIMALRQGGLVMRNYRLIEATLYVTFEPCIMCAGAMIHSRIGRVVFGVRNSKRGAAGSLMNVLNYPGMNHRVEITEGILADECAALLCDYYRMPRRVFNAQKRAQSSINSGGSSDGGSGSETPGTSESATPKNSGGSSGGSAKNTITKALKLRIVRPYNSAEVEKIVADEKNNRERIALEKNKDKVKEACSKHLKVAAYCTTQVERNACLFCKARKLDDKFYQKLRGQFPDAVFWQEIGEIFRQLQKQAAEIYNQSLIELYYEILIKGKGFANASSVEHYLSDVCYTRAAELFKNAAIASGLRGKVKSNFRLKELKNMRSGLPTTKSDNFPIPLVKQKGGQYAGFEISSHNDDFIIKIPFGRWQVKKEIDKYRPWEKFDFEQVRKSPKPISLLLSTQRRKRNKGWSKDEGTEAEIRKVMNGDYQTSYIEVKRGSKIGEKSAWMLNLSIDVPKIDKGVDPSIIGGIDVGVKSPLVCAINNALSRYSIGDNDLFHFNKKMFARRRILLRKNRHKRAGHGARNKLKPITVLTEKSERFRKKLIERWACEIANFFIKNKVGTVQMENLESMKRRGDSYFNIRLRGFWPYAEMQNKIEFKLKQYGIEIRRVAPNNTSRTCSKCGHLNNYFNFEYRKKNKFPHFKCEKCYFKEDADYNAALNISNPRLKSTKEEP

SEQ ID NO: 2012 - protein, 726 aa, synthetic construct
SEVEFSHEYWMRHALTLAKRARDEREVPVGAILVLNNRVIGEGWNRAIGLHDPTAHAEIMALRQGGLVMQNYRLIDATLYVTFEPCVMCAGAMIHSRIGRVVFGVRNNKHGAAGSLVNVLNYPGMNHRVEITEGILADECAALLCDFYRMPRQVFNAQKKAQSSINSGGSSGGSSGSETPGTSESATPESSGGSSGGSAKNAITKTLKLRIVRPYNSAEVEKIVADEKNNREKIALEKNKDKVKEACSKHLKVAAYCTTQVERNACLFCKARKLDDKFYQKLRGQFPDAVFWQELGEIFRQLQKQAAEIYNQSLIELYYEIFIKGKGFANASSVEHYLSDVCYTRAAELFKNAAIASGLRGKVKSNFRLKELKNMKSGLPTTKSDNFPIPLVKQKGGQYTGFEISGHNDDFIIKIPFGRWQVKKEIDKYRPWEKFDFEQVRKSPKPISLLLSTQRRKRNKGWSKDEGTEAEIRKVMNGDYQTSYIEVKRGSKTGEKSAWMLNLSIDVPKIDKGVDPSIIGGIDVGVKSPLVCAINNAFSRYSISDNDLFHYNKKMFARRRILLKKNRHKRAGHGAKNKLKPISILTEKGKRFRKKLIERWACEIADFFIKNKVGTVQMENLESMKRKEDSYFNIRLRGFWPYAEMQNKIEFKLKQYGIEIRKVAPNNTSKTCSKCGHLNNYFNFEYRRTNKFPHFKCEKCNFKENADYNAALNISNPKLKSTKEES

SEQ ID NO: 2013 - protein, 726 aa, synthetic construct
SEVEFSHEYWMRHALTLAKRARDEREVPVGAVLVLNNRVIGEGWNRTTGLHDPTAHAEIMALRQGGLVMQNHRLVDATLYVTFEPCVMCAGAMIHSRIGRVVFGVRNSKRGAAGSLTNVLNYPGMNHRVEITEGILVDECAALLCDFYRMPRQVFNAQRKAQSTINPGGSSGGSSGSETPGASESVTPKSSGGSSGGSAKNTITKTLKLRIVRPYNSAEVEKIVADEKNNREKIALEKNKGKVKEACSKHLEVAAYCTTQVERNACLFCKARKLDDKFYQKLRGQFPDAVFWQELGEIFRQLQKQAAEIYNQSLIELYYEIFIKGKGITNASRVEHYLSDVCYTRAAELFKNAAIASGLRSKVRSNFRLKELKNMKSGLPTTKSDNFPIPLVKQKGGQYTGFEISNHNSDFIIKIPFGRWQVKEEINKYRPWEKFDFEQVRKSPKPISLLLSTQRRKRNKGWSKDEGTEAEIRKVMNGDYQTSYIEVRRGNKIGERSAWMLNLSIDVPKIDKGVNPSIIGGIDVGVRSPLVCAINNAFSRYSISDNDLFRFNKKMFARRRILLGKNRHKRAGHGVKNKLKPITILTEKSGRFRKKLIERWACEIADFFIKNKVGTVQMENLESMKRKEDSYFNIRLRGFWPYAEMQNKIEFKLKQYGIKIRKVAPNNTSRTCSECGHLNNYFSFEYRKKNKFPHFKCEKCNFKEDADYNAALNISNPKLKGTKEEL

SEQ ID NO: 2014 - protein, 726 aa, synthetic construct
SEVEFSHEYWMRHALTLAKRARDEREVPVGAVLVLNNRVIGEGWNRAIGLHDPTAHAEIMALRQGGLVMQNYRLSDATLYVTFEPCVMCAGAMIHSRIGRVVFGVRNSKRGAAGSLMNILNYPGMNHRVEITEGILADECAALLCDFYRMPRQVFNAQKKAQSSINSGGSSGGSSGSETPSTSESATPESSGGSSGGSAKNTITKTLQLRIVRPYNSAEVEKIVADEKNSREKIALEKNKDKVKEACGKHLKMASYCTTQVERNACLFCKARKLDDKFYQKLRGQFPDAVFWQELGGIFRQLQKQAAEIYNQSLIELYYEIFIKGKGITNASRVEHYLSDVCYTRAAELFKNAAIASGLRGKVKSNFRLKELKNMKSGLPTTKSDNFPIPLVKQKGGQYAGFEISSHNDDFIIKIPFGRWQVKKEIDKYRPWEKFDFEQVRKSPKPISLLLSTQRRKRSKGWSEDEGTEAEIKKVMNGDYQTSYIEVKRGSKIGEKSAWMLNLSIDVPKIDKGVDPSIIGGIDVGVKSPLVCAISNAFSRYSISDNDLFHFNKKMFARRRILLKKSKHKRAGHGAKNKLKPITILTEKSRRFRKKLIERWACEIADFFIKNKVGTVQMENLESMKRKEDSYFNIRLRGFWPYAEMQNKIEFKLKQYGIEIRKVAPNNTSKTCSKCGHLNNYFNFEYRKKNKFPHFKCEKCNFKENADYNAALNISNPKLKSTKGEP

SEQ ID NO: 2015 - protein, 726 aa, synthetic construct
SEVEFSHEYWMRHALTLAKRARDEREVPVGAVLVLNNRVIGEGWNRAIGLHDPTAHAEIMALRQGGLVMQNYRLVDATLYVTFEPCVLCAGAMVHSRIGRVVFGVRNSKRGAAGSLMNVLNYPGMNHRVEITEGILADECAALLCDFYRMPRQVFNAQKKARSDISSGGSSGDSSGSETPGTRESPTPGSSGGSSGGSAKNTITKTLKLRIVRPYNSAEVEKIVADEKNNREKTALEKNKDKVKEACSEHLKVATYCTTQVERNACLFCKARKLDDKFYQKLRGQFPDAVFWQELGEILRQLQKQAAEIYNQSLVELYYEIFIKGRGFANASSVEHYLSDVCYTRAAELFKNAAIASGLRGKVKSNFRLKELKNMKSGLPTTRSDNFPIPLVKQKGGQYTGFEISSHNDDFIIKIPFGRWQVKKEIVKYRPWEKFDFEQVRKSPKPISLLLSTQRRKRNKGWSKDEGTEAEIRKVMNGDYQTSYIEVKRGSKTGEKSAWMLNLSIDVPKIDKGVDPSIIGGIDVGVKSPLVCAINNAFSRYSISDNDLFRFNKKMFARRRILLRKNRHKRAGHGAKNKLKPISILTGKSERFRKKLIERWACEIADFFIKNKVGTVQMENLESMKRKEDSYFNIRLRGFWPYAEMQNKIEFKLKQYGIEIRKVAPNNTSKTCSKCGHLNNYFNFEYRKKNKFPHFKCEKCNFKENADYNAALNISNPKLKNTMEEP

SEQ ID NO: 2016 - protein, 725 aa, synthetic construct
SEVEFSHEYWMRHALTLAKRARDEREVPVGAVLVLNNRVIGEGWNRAIGLHDPTAHAEIMALRQGGLVMQNYRLTDATLYVTFEPCVMCAGAMIHSRIGRVVFGVRNSKRGAAGSLMNVLNYPGMNHCVEITEGILVDECAALLCDFYRMPRQVLNAQKKAQSSISSGGSSGGSSGSVTPGASGSVTPSSGGSSGGSAKNTITKTLKLRIVRPYNSAEVEKIVADEKSNREKIALEKNKDKVKEACSEHLKVAAYCTTQVERSACLFCKARKLDDKFYQKLRGQFPDAVFWQEIGEIFRQLQKQAAEIYNQSLIELYYEIFIKGKGFANASSVEHYLSDVCYTRAAELFKNAAIASGLRGKVKSNFRLKELKNMKSGLPTTKSDNFPIPLVKQKGGQYTGFEISSHDDDFVIKIPFGRWQVKKEIDKYRPWEKFDFEQVRKSPKPISLLLSTQRRKRNKGWSRDEGTEAEIRKVMNGDYQTSYIEVKRGSKIGEKSAWMLSLSIDVPKIDKGVDPSIIGGIDVGVKSPLVCAINNALSRYSIDDNDLFHFNKKMFARRRILLKRNRHKRAGHGAKNKLKPITILTEKSRRFRKKLIERWACEIADFFIKNKVGTVQMENLESMKRREDSYFNIRLRGFWPYAEMQNKIEFKLKQYGIEIRKVAPINTSKTCSKCGHLNNYFNFEYRKKNKFPHFKCEKCNFKENADYNAALNISNPKLKGTKEEP

SEQ ID NO: 2017 - protein, 726 aa, synthetic construct
SEVEFSHEYWMRHALTLAKRARDEREVPVGAILVLNNRVIGEGWNRAIGLHDPTAHAEIMALRQGGLVMQNYRLIDATLYVTFEPCVMCAGAMVHSRIGRVVFGVRNSKRGAAGSLMNVLNYPGMNHCVEITEGILVDECAALLCDFYRMPRLVLNAQKKAQSSISPGGSSGGSSGSETPGASGSVIPKSSGGSSAGSTKDTITKTLKLRIVRPYNSAEVEKVVADEKNNREKIAMEKNKDKVKEACSKHLKVASYCTTQVERNACLFCKARKLDDKFYQKLRGQFPDAVFWQELGGIFRQLQKQAAEIYNQSLIELYYEIFIKGKGITNASRVEHYLSDVCYTRAAELFKNAAIASGLRSKVRSNFRLKELKNMKSGLPTTKSDNFPIPLVKQKGGQYTGFEISSHNSDFIIKIPFGRWQEKEEIDKYRPWEKFDFEQVRKSPKPISLLLSTQRRKRNRGWSKDEGTEAEIKKVMNGDYQTSYIEVMRGSKIGEKSAWMLNLSIDVPKIDKGVDPSIVGGIDVGVKSPLVCAINNAFCRYSISDNDLFHFNKKMFARRRILLKKNGHKRAGHGAKNKLKPITIMTEKSKRFRKKLIERWACEIADFFVKNKVGTVQMENLESMKRKEDSYFNIRLRGLWPYAEMQNKIEFKLKQYGIVVRKVAPNNTSKTCSKCGHLNNYFNFEYRKKNKFPHFKCEKCNFKENADYNAALNISNPKLRSTKEEP

SEQ ID NO: 2018 - protein, 726 aa, synthetic construct
SEVEFSHEYWMRHALTLAKRARDEREVPVGAVLVLNNRVIGEGWNRAIGLHDPTAHAEIMALRQGGLVMQNYRLIDATLYVTFEPCVMCAGAMVHSRIGRVVFGVRNSKRGAAGSLMNVLNYPGMNHRVEITEGILADECAALLCDFYRMPRQVFNARKKARSNINSGGSSGGSSSSEAPGTSGSATPKSSGGSSGGSVKNTITKTLKLRIVRPYNSAEVERIVADEKNNREKIALEKNKDKVKEACSKHLKVASYCTTQVERNACPFCKARKLDDKFYQKLRGQFPDAVFWQELGEILRQLQKQAAEIYNQSLIELYYEIFIKGKGIANASSVEHYLSDVCYTRAAELFKNAAIASGLRNKIKSNFRLKELRNMKSGLPTTKSDNFPIPLVRQKGGQYTGFEISNHNGDFIIKIPFGRWQVKKEICKHRPWEKFDFEQVRKSPKPISLLLSTQRRKRNKGWGKDEGTEAEIRKVMNGDYQTSYIEVKRGSKIGEKSAWMLNLSIDVPKIDKGVDPSINGGIDVGVKSPLVCAINNALSRYSISDNDLFHFNKKMFARRRILLRKNRHKRAGHGARNKLKPISVLTGKSERFRKKLIERWACEIADFFIKNKVGTVQMENLESMKKKEDSYFNIRLRGFWPYAEMQNRIEFKLRQYGIEVRKVAPNNTSKTCSKCGHLNNYFNFEYRKKNKFPHFKCEKCNFKENADYNAALNISNPKLKSTKEEP

SEQ ID NO: 2019 - protein, 726 aa, synthetic construct
SEVEFSHEYWMRHALTLAKRARDEREVPVGAILVLNNRVIGVGWNRAIGQHDPTAHAEIMALRQGGLVMQNYRLIDATLYVTFEPCVMCAGAMIHSRIGRVVFGVRNSKHGAAGSLVNVLNYPGMNHRVETTEGILAEECAALLCDFYRMPRQVFNAQKKAQSTINSGSSSGGSSGSETPGTSESPAPESSGGSSGSSAKNTITKTLKLRIVRPYNSAEVEKIVADEKNNREKIALEKNKDKVKEACSKHLKVAAYCTTQVERNACLFCKARKLDDKFYQKLRGQFPDAVFWQEIGEIFRQLQKQAAEIYNQSLIELYYEIFIKGKGFANASSVEHYLSDVCYTRAAELFKNAAIASGLRGKVKSNFRLKELKNMKSGLPTTKSDNFPIPLVKQKGGQYTGFEISSHNDDFIIKIPFGRWQMKKEIDRYRPWEKFDFEQVRKSPKPISLLLSTQRRKRNKGWGKDAGTEAEIRKVMNGDYQTSYIEVKRGSKIGEKSVWMLNLSIDVPKIDKGVDPSIIGGIDVGVKSPLVCAINNTSDRYGISDNDLFHFNKKMFARRRILLKKNGHRRAGHGAKNKLKPITVLTKKSERFRKKLIERWACEIADFFIKNKVGTVQMENLESLKRKEDSYFNIRLRGFWPYAEMQNKIEFKLKQYGIEIRKVAPNNTSKTCSKCGHLNSYFNFEYRKKNKFPHFKCEKCNFKENADYNAALNISNPKLKSTKEEP

SEQ ID NO: 2020 - protein, 726 aa, synthetic construct
SEVEFSHEYWMRHALTLARRARDEREVPVGAVLVLNNRVIGGGWNRAIGLHDPTAHAEIMALRQGGLVMQSCRLVDATLYVTFEPCVMCAGAMIHSRIGRVVFGVRNSKRGAAGSLMNVLNYPGMNHRVEITEGILAGECAALLCDFYRMPRQVFNAQKKAQSTINSGGSSGGSSSSETPGTSGSATPEGSGGSSGGSAKNTITKTLKLRIVRPYNSAEVEKIVADEKNNREKIALEKNKGKVREACNKHLKVASYCTTQVERNACPFCKARKLDDKFYQKLRGQFPDAVFWQELGEILRQLQKQAAEIYNQSLIELYYEIFIKGRGFANASSVEHYLSDVCYTRAAELFKNAAIASGLRGKVKSNFRLKELKNMKSGLPTTKSDNFPIPLVKQKGGQYTGFEISSHNDDFIIKIPFGRWQVKKEIDKYRPWEKFDFEQVRKSPKPISLLLSTQRRKRNKGWSKDEGTEAEIRKVMNGDYQTSYIEVKRGSKIGEKSAWMLNLSIDVPKIDKGVDPSIIGGIDVGVKSPLVCAINNALSRYSISDNDLFHFNKKMFARRRILLRKNRHKRAGHGAKNKLKPITMMTEKSKRFRKKLIERWAREIADFFIKNKVGTVQMENLESMKRKEDSYFNIRLRGFWPYAEMQDKIEFKLKQYGIVVRKVAPNNTSKTCSKCGHLNNYFNFEYRRKNKFPHFKCEKCNFKENADYNAALNICNPRLKGTKEEP

SEQ ID NO: 2021 - protein, 726 aa, synthetic construct
SEVEFSHEYWMRHALTLARRARDEREVPVGAVLVLNNRVIGEGWNRTTGLHDPTAHAEIMALRQGGLVMRNYRLTDATLYVTFEPCVMCAGAMIHSRIGRVVFGVRNSKRGAAGSLMNVLNYPGMNHCVEITEGILVDECAALLCDFYRMPRQVLNAQKKAQSSISPGGSSGGSSGSGTPGASESVTPKSSGGSSGGSAKDIITKTLKLRIVRPYNSAEVEKIVADEKNNREKIALEKNKDKVKEACSKHLKVASYCTTQVERNACLFCKARKLDDKFYQKLRGQFPDAVFWQELGEIFRQLQKQAAEIYNQSLIELYYEIFIKGKGFANASSVEHYLSDVCYARAAELFKNAAIASGLRGKVKSNFRLKELKNMKSGLPTTKSDNFPIPLVKQKGGQYTGFEISSHNDDFVIKIPFGRWQVRKEIDKYRPWEKFDFEQVRKNPKPISLLLSTQRRKRNKGWSKDEGTEAEIRRVMNGDYQTSYIEVKRGSKIGEKSAWMLNLSIDVPKVDKGVDPSIIGGIDVGVKSPLVCAINDAFSRYSISDNDLFHFNKKMFARRRILLKKNRHQRAGHGAKNKLKPISILTEKSKRFRKKLIERWACEIADFFIKNKVGTVQMENLESMKRKEDSYFNIRLRGFWPYAEMQNKIEFKLKQYGIEIRKVAPNNTSKTCSKCGHLNNYFSFEYRRKNRFPHFKCEKCNFKENADYNAALNISNPKLKSTKEEP

SEQ ID NO: 2022 - protein, 726 aa, synthetic construct
SEVEFSHEYWMRHALTLAKRARDEREVPVGAVLVLNNRVIGEGWNRAIGLHDPTAHAEIMALRQGGLVMQNYRLVDATLYVTFEPCVLCAGAMVHSRIGRVVFGVRNSKRGAAGSLMNVLNYPGMNHRVEITEGILADECAALLCDFYRMPRQVFNAQKKARSNINSGGSSGGSSGSETPGASESVTPKSSGGSSGGSAKNTITKTLKLRIVRPYNSAEVEKIVADEKNNREKIALEKNKDKVKEACSKHLKVASYCTTQVERNACPFCKARKLDDKFYQKLRGQFPDAVFWQELGEILRQLQKQAAEIYNQSLIELYYEIFIKGRGFANASIVEHYLSDVCYTRAAELFKNAAIASGLRGKVKSNFRLKELRNMKSGLPTTKSDNFPIPLVRQKGGQYTGFEISNHNGDFIIKIPFGRWQVKKEINKFRPWEKFDFEQVRKSPKPISLLLSTQRRKRNKGWSRDEGTEAEIRKVMNGDYQTSYIEVKRGSKIGEKSAWMLNLSIDVPKIDKGVDPSIIGGIDVGVKSPLVCAINNASSRYSISDNDLFRFNKKMFARRRILLKKNRHKRAGHGAKNKLKPISILTEKSERFRKKLIEKWACEIADFFVKNKVGTVQMENLESMKRKEDSYFNIRLRGFWPYAEMQNKIEFKLKQYGIKVRKVAPNNTSKTCSKCGHLNNYFSFEYRKKNKFPHFKCEKCNFKENADYNAALNISNPKLKSTKEEP

SEQ ID NO: 2023 - protein, 726 aa, synthetic construct
SGDEFSHEYWMRHALTLAKRARDGREVPVGAVLVLNNRVIGEGWNRAIGLHDPTAHAEIMALRQGGLVMQNYRLIDATLYVTFEPCVMCAGAMVHSRIGRVVFGVRNSKRGAAGSLVNVLDYPGMNHRVEIMEGILTDECAALLCDFYRMPHQVLNAQKKAQSSINSGGSSGGSSGSETPGTSGSATPEGSGGSSGGSTKNTITKTLKLRIVRPYNSAEVEKIVADEKNNREKIALEKNKGKVKEACSKHLKVATYCTTQVERNACLFCKARKLDDKFYQKLRGQFPDAVFWQEVGEIFRQLQKQAAEIYNQSLIELYYEIFIKGKGIANASSVGHYLSDVCYTRAAELFKNAAIASGLRGKIKSNFRLKELRNMKSGLPTTKSDNFPIPLVKQKGGQYTGFEISNHNGDFIIKIPFGRWQAKKEIDKYRPWEKFDFEQVRKSPKPISLLLSTQRRKRNRGWSKDEGTEAEIRKVMNGDYQTSYVEVKRGSKIGEKSAWMLNLSIDVPKIDKGVDPGIIGGIDVGVKSPLVCAINNASSRYSISDNDLFHFNKKMFARRRILLKKNRHKRAGHGAKNKLKPITIMTEKSKRFRKKLIERWACEIADFFIKNKVGTVQMENLESMKRKEDSYFNIRLRGFWPYAEMQNKIEFKLKQYGIEIRKVAPNNTSKTCSKCGHLNYYFNFEYRKKNKFPHFKCEKCNFKEDADYNAALNISNPKLKSTKEEP

SEQ ID NO: 2024 - protein, 726 aa, synthetic construct
SEVEFSHEYWMRHALTLAKRARDEREVPVGAVLVLNNRVIGEGWNRAIGLHDPTAHAEIMALRQGGLAMQNYRLVDATLYVTFEPCVLCAGAMVHSRIGRVVFGVRNSKRGAAGSLMNVLNHPGMNHRVEITGGILADECAALLCDFYRMPRQVFNAQKKARSNINSGGSSGGSSGSETLGTSESATPENSGGSSGGSAKNTITKTLKLRIVRPYNSAEVEKIVADEKNNREKVALEKNKDKVKEACSEHLKVAAYCTTQVERNACLFCKARKLDDKFYQKLRGQFPDAVFWQEIGEIFRQLQKQAAEIYNQSLIELYYEIFIKGRGFANAGSVEHYLSDVCYTRAAELFKNAAIASGLRGKVKSNFRLKELKNMKSGLPTTKSDNFPIPLVKQKGGQCTGFEISSHNDDFIIKIPFGRWQVKKEIDKYRPWEKFDFEQVRKSPKPISLLLSTQRRKRYKGWSKDEGTEAEIRKVMNGDYQTSYIEVKRGSKTGEKSAWMLNLSIDVPKIDKGVDPSIIGGIDVGVKSPLVCAINNAFSRYSISDNDLFHYNKKMFARRRILLKKNRHKRAGHGAKNKLKPISILTEKSKRFRKKLIERWACEIADFFIKNKVGTVQIENLESMKRKEDSYFNIRLRGFWPYAEMQGKIEFKLRQYGIVVRKVAPNNTSKACSKCGHLNNYFNFEYRKKNKFPHFKCEKCNFREDADYNAALNISNPKLKSTKEEP

SEQ ID NO: 2025 - protein, 726 aa, synthetic construct
SEVEFGHEYWMRHALTLAKRARDEREVPVGAVLVLNNRVIGVGWNRAIGLHDPTAHAEIMALRQGGLVMQNHRLVDATLYVTFEPCVMCAGAMIHSRIGRVVFGVRNSKRGAAGSLTNVLNYPGMNHRVEITEGILVDECAALLCDFYRMPRQVFNAQKKAQSTINSGGSSGGSSGSETPGTSESATPKSSGGSSGGSAKNTITKTLQLRIVRPYNSAEVEKIVADEKNNRERIALEKNKDKVKEACSKHLKVAAYCTTQVERNACLFCKARKLDDRFYQKLRGQFPDAVFWQEIGEIFRQLQRQAAEIYNQSLIELYYEIFIKGKGFANASSVEHYLSDVCYTRAAELFKNAAIASGLRGKVKSNFRLKELKNMKSGLPTTKSDNFPIPLVKQKGGQYTGFEISSHNDDFIIKIPFGRWQAKKEIDKYRPWEKFDFEQVRKSPKPISLLLSTRRRKRNKGWSKDEGTEAEIRRVMNGDYQTSYIEVKRGSKIGEKSAWMLNLSIDVPKIDKGVDPSIIGGIDVGVKSPLVCAINNAFSRYSISDNDLFHFNKKMFARRRILLKKNRHQRAGHGAKNKLKPITILTEKSGRFRKKLIERWACEIADFFIKNKVGTVQMENLESMKRKEDSYFNIRLRGFWPYAEMQNKIEFKLKQYGIKIRKVAPNNTSKTCSKCGHLNNYFSFEYRKKNKFPHFKCEKCNFKENADYNAALNISNPKLMSTKEEP

SEQ ID NO: 2026 - protein, 726 aa, synthetic construct
SEVEFSHEYWMRHALTLAKRARDEREVPVGAVLVLNNRVIGEGWNRAIGLHDPTAHAEIMALRQGGLVLQNYRLIDATLYVTFEPCVMCAGAMIHSRVGRVVFGVRNSKHGAAGSLVNVLDYPGMGHRVEITEGILADECAALLCDFYRMPRQVFNAQKRAQSSINSGGSSGGNSGSETPGTSESVTPESSGGGSSGSAKNTITKTLQLRIVRPYNSAEVEKIVADEKNNREKIALEKNKDKVKEACSKHLKVASYCTTQVERNACPFCKARKLDDKFYQKLRGQFPDAVFWQELGEILRQLQKQAAEIYNQSLIELYYEIFIKGRGFANAGGVEHYLSDVCYTRAAELFKNAAIASGLRGKVKSNFRLKELKNMKSGLPTTKSDNFPIPLVKQKGGQYTGFEISSHNDDFIIKIPFGRWQVKKEIDKYRPWEKFDFEQVRKSPKPISLLLSTQRRKRNKGWSKDEGTEAEIRKVMNGDYQTSYIEVKRGSKTGEKSAWMLNLSIDVPKIDKGVDPSIIGGIDVGVKSPLVCAINNAFSRYSISDNDLFRFNKKVFARRRILLKKNRHKRAGHGTKNKLKPITILTEKSGRFRKKLIERWACEIANFFVKNKVGTVQMEDLESMKRKEDSYFNIRLRGFWPYAEMQNKIEFKLKQYGIKIRKVAPNNTSKTCSKCGHLNNYFNFEYRKKNKFPHFKCEKCNFKEDADYNAALNISNPKLKSTKEEP

SEQ ID NO: 2027 - protein, 726 aa, synthetic construct
SEDEFSHEYWMRHALTLAKRARDGREVPVGAVLVLNNRVIGEGWNRAIGLHDPTAHAEIMALRQGGLVMQNYRLIDATLYVTFEPCAMCAGAMVHSRIGRVVFGVRNGKRGAAGSLMNVLNYPGMNHRVEITEGILADECAALLCDFYRMPRRVFNAQKKAQSSINSGGSSGGGSGSETPSTSENTTPESSGGSSGGPAKNTITKTLKLRIVRPYNSAEVEKIVADEKNNREKTALERNKDKVKEACSKHLKVAAYCTTQVERNACLFCKARKLDDKFYQKLRGQFPDAVSWQEIGEIFRQLQKQAAEIYNQSLIELYYEIFIKGKGFANASSVEHYLSDVCYTRAAELFKNAAIASGLRGKVKSNFRLKELKNMKSGLPTTKSDNFPIPLVKQKGGQYTGFEISSHNDDFIIKIPFGRWQVKKEIDKYRPWEKFDFEQVRKSPKPISLLLSTQRRKRNKGWSKDEGTEAEIKKVMNGDYQTSYIEVKRGSKIGEKSAWMLNLSIDVPKIDKGVDPRIIGGIDVGVKSPLVCAINNAFSRYSISDNDLFRFNKKMFARRRILLKKNRHKRAGHGAKNKLKPISILTEKSKRFRKKLIERWACEIADFFIKNKVGTVQMENLESMKRKEDSYFNIRLRGFWPYAEMQSKIEFKLKQYGIKIRRVAPNNTSKTCSKCGHLNNYFNFEFRKKNKFPHFKCEKCNFKEDADYNAALNISNPKLKGTKEEP

SEQ ID NO: 2028 - protein, 726 aa, synthetic construct
SEVEFSHEYWMRHALTLAKRARDEREVPVGAVLVLNNRVIGEGWNRAIGLHDPTAHAEIMALRQGGLVMQNYRLSDATLYVTFEPCVMCAGAMIHSRIGRVVFGVRNSKRGAAGSLMNVLNYPGMNHCVEITEGILADECAALLCDFYRMPRQVFNAQKKAQSSINSGGSSGGSSGSETPSTSESATPESSGGSSAGSTRDTITKTLKLRIVRPYNSAEVEKIVADEKNSREKIALEKNKDKVKEACSEHLKVATYCTTQVERNACLFCKARKLDDKFYQELRGQFPDAVFWQEIGEIFRQLQKQAAEIYNQSLIELYYEIFIKGKGIANASSVGHYLSDVCYTRAAELFKNAAIASGLRSKIKSNFRLKELRNMRGGLPTTKSDNFPIPLVKQKGGQYTGFEISSHNDDFIIKIPFGRWQVKKEINKHRPWEKFDFEQVRKSPKPISLLLSTQRRKRNKGWSKDEGTEAEIRKVMKGDYQTSYIEVKRGSKIGEKSAWMLNLSIDVPKIDKGVDPGIIGGIDVGVKSPLVCAINNATSRYSISDNDLFHFNKKMFARRRILLKKNRHKRAGHGAKNKLKPITIMTEKSKRFRKKLIERWACEIADFFIKNKVGTVQMENLESMKRKEDSYFNIRLRGFWPYAEMQNKIEFKLRQYGIEIRKVAPNNTSKTCSKCGHLNNYFNFEYRKKNKFPHFRCEKCNFKENADYNAALNISNPKLKSTKEEP

SEQ ID NO: 2029 - protein, 726 aa, synthetic construct
SEVEFSHEYWMRHALTLARRARDEREVPVGAVLVLNNRVIGEGWNRAIGLQDPTAHAEIMALRQGGLVMQNYRLSDATLYVTFEPCVMCAGAMIHSRIGRVVFGVRNSKRGAAGSLMNVLNYPGMNHCVEITEGILVDECAALLCDFYRMPRQVLSAQKKAQSSVSSGGSSGGSSGSETPGASGSVTPKSSVGSSAGSAKNTITKTLKLRIVRPYNSAKVEKIVADEKNNREKIALEKNRDKVKEACSKHLKVAAYCTTQVERNACLFCKARKLDDKFYQKLRGQFPDAVFWQEISEIFRQLQKQAAEIYNQSLIELYYEIFIKGKGFANASSVEHYLSDVCYTRAAELFKNAAIASGLRGKVKSNFRLKELKNMKSGLPTTKSDNFPIPLVKQKGGQYTGFEINSHNDDFIIKIPFGRWQVKKEVDKYRPWEKFDFEQVRKSPKPISLLLSTQRRKRNKGWSKDEGTEAEIRKVMNGDYQTSYIEVKRGSKIGEKSAWMLNLSIDVPKIDKGVDPSIIGGIDVGVKSPLVCAINNAFSRYSISDNDLFHFNKKMFARRRILLKKNRHRRAGHGAKNKLKPIAVLAEKSEGFRKKLIERWACEVADFFIKNKVGTVQMENLESMKRREDSYFNIRLRGFWPYAEMQNKIEFKLRQYGIEIRKVAPNNTSKTCSKCGHLNNYFDFEYRKKNKFPHFKCEKCNFKENADYNAALNISNPKLRSTKEEP

SEQ ID NO: 2030 - protein, 726 aa, synthetic construct
SEVEFSHEYWMRHALTLAKRARDEREVPVGAILVLNNRVIGEGWNRAIGLHDPTAHAEIMALRQGGLVMQNYRLIDATLYVTFEPCVMCAGAMIHSRIGRVVFGVRNSKHGAAGSLVNVLNYPGMNHRVEITEGILADECAALLCDFYRMPRQVFGARRKAQSSINPGGSTGGSSGSETPGASESVTPKSSGGSPAGSTKNTITKTLKLRIVRPYNSAEVEKIVADEKNNREKIALERNKDKVREACNKHLKVAAYCTTQVERNACLFCKARKLDDKFYQKLRGQFPDAVFWQELGEILRQLQKQAAEIYNQSLIELYYEIFIKGRGFANASNVEHYLSDVCYTRAAELFKNAAIASGLRGKVKGNFRLKELKNMKSGLPTTKSDNFPIPLVKQKGGQYTGFEISSHNDDFIIKIPFGRWQVKKEIDKYRPWEKFDFEQVRRSPKPISLLLSTQRRKRNKGWSKDEGTEAEIRKVMNGDYQTSYIEVKRGSKTGEKSAWMLNLSIDVPKIDKGVDPSIIGGIDVGVKSPLVCAINNAFGRYSISDNDLFHFNKKMFARRRILLRKNRHKRAGHGAKNKLKPISILTGKSERFRKKLIERWACEIADFFIKNKVGTVQMENLESMKRKEDSYFNIRLRGFWPYAEMQSKIEFKLKQYGIEIRKVAPNNTSKTCSKCGHLNNYFNFEYRKKNKFPHFKCEKCNFKENADYNAALNISNPKLKSTKEEP

SEQ ID NO: 2031 - protein, 726 aa, synthetic construct; identical to SEQ ID NO: 684

SEQ ID NO: 2032 - protein, 726 aa, synthetic construct
SEVEFSHEYWMRRALTLAKRARDEREVPVGAVLVLNNRVIGEGWNRAIGLHDPTAHAEIMALRQGGLVMQNYRLIDATLYVTFEPCVMCAGAMIHSRIGRVVFGVRNNKRGAAGSLMNVLNYPGMNHRVEITEGILADECAALLCDFYRMPRQVFNAQKKAQSSINSGGSSGGSSGSETPGTSESATPESSGGSSGGSTKNTITKTLQLRIVRPYNSAEVEKIVAAEKDSREKIALEKNKDKVKEACSKHLKVASYCTTQVERNACPFCKARKLDDKFYQKLRGQFPDAVFWQELGEIFRQLQRQAAEIYNQSLIELYYEIFIKGKGFANASSVEHYLSDVCYTRAAELFKNAAIASGLRGKVKSNFRLKELKNMKSGLPTTKSDNFPIPLVKQKGGQYTGFEISSHNDDFIIKIPFGRWQVKKEIDKYRPWEKFDFEQVRKSPKPISLLLSTQRRKRNKGWSKDEGTEAEIRKVMNGDYQTSYIEVKRGSKIGEKSAWMLNLSIDVPKIDKGVDPSIIGGIDVGVKSPLVCAINNALSRYSISDNDLFHFNKKMFARRRILLRKNRHKRAGHGAKNKLKPITIMTEKSKRFRKKLIERWACEIADFFIKNKVGTVQMENLESMKRREDSYFNIRLRGFWPYAEMQDRIEFKLKQYGIEIRRVAPNNTSRTCSKCGHLNNYFNFEYRKKNKFPHFKCEKCNFREDADYNAALNISNPKLKSTKEEP

SEQ ID NO: 2033 - protein, 726 aa, synthetic construct
SEVEFSHEYWMRHALTLAKRARDEREVPVGAVLVLNNRVIGEGWNRAIGLHDPTAHAEVMALRQGGLVMQNYRLTDATLYVTFEPCVMCAGAMIYSRIGRVVFGVRNSKRGAAGSLMNVLNYPGMNHCVEITEGILVDECAALLCDFYRMPRQVLNAQKKAQSSISPGGSSGGSSGSETLGTSESATPESSGGSSGGSAKNTITKALKLRIVRPYNSAEVEKIVADEKNNRERIALEKNKDKVKEACSKHLKVAAYCTTQVERNACLFCKARKLDDKFYQKLRGQFPDAVFWQEIGEIFRQLQKQAAEIYNQSLVELYYEIFIKGKGIANASSVEHYLSDVCYTRAADLFKNAAIASGLRGKVKGNFRLKELKNMKSGLPTTKSDNFPIPLVKQKGGQYTGFEISSHNDDFIIKIPFGRWQVKKEIDKYRPWEKFDFEQVRKSPKPISLLLSTQRRKRNKGWSKDEGTEAEIRKVMNGDYRTSYIEVKRGSKTGEKSAWMLNLSIDVPKIDKGVDPSIVGGIDVGVKSPLVCAINNALSRYSISDNDLFHFNKKMFARRRILLKKNRHKRAGHGAKNKLRPISILTGKSERFRKKLIERWACEIADFFIKNKVGTVQMENLESMKRREDSYFNIRLRGFWPYAKMQNKIEFKLKQYGIEIRKVAPNNTSKTCSKCGHLNNYFSFEYRKRNKFPHFKCEKCNFKEDADYNAALNISNPKLKSTKEEP

SEQ ID NO: 2034 - protein, 726 aa, synthetic construct
SEVEFSHEYWMRRALTLAKRARDEREVPVGAVLVLNNRVIGVGWNRAVGLHDPTAHAEIMALRQGGLVMQNYRLIEATLYVTFEPCIMCAGAMIHSRIGRVVFGVRNSKRGAAGSLMNVLNYPGMNHRVEITEGILADECAALLCDYYRMPRQVFNARKKVQSSINSGGSSDGGSSSETPGTSESATPESSGGSSGGSAKNTITKTLKLRIVRPYNSAEVEKIVADEKNNREKIALEKNKDKVKEACSEHLKVAAYCTTQVERNACLFCKARKLDDKFYQKLRGQFPDAVFWQELGEIFRQLQKQAAEIYNQSLIELYYEIFIEGKGSANARSVEHYLSDVCYTRAAELFKNAAIASGLRGKVKGNFRLKELKSMKSGLPTTKSDNFPIPLVKQKGGQYTGFEISSHDDDFIIKIPFGRWQVKKEIDKYRPWEKFDFEQVRKSPKPISLLLSTQRRKRNKGWSKDEGTEAEIRKVMNGDYQISYIEVKRGSKIGEKSAWMLSLSIDVPKIDKGVDPSIIGGIDVGVRSPLVCAIDNAFSRYSISDNDLFHFNKKMFARRRILLKKNRHKRVGHGAKNKLKPISILTEKSKRFRKKLIERWACEIADFFIKNKVGTVQMENLVSMKRKEDSYFNIRLRGLWPYAEMQNKIEFKLKQYGIEIRKVAPNNTSKTCSKCGHLNSYFNFEYRRKNKFPHFKCEKCNFKENADYNAALNISNPKLKSTKEEP

SEQ ID NO: 2035 - protein, 726 aa, synthetic construct
SEVEFSHEYWMRHALTLAKRARDEREVPVGAILVLNNRVIGEGWNRAIGLHDPTAHAEIMALRQGGLVMQNYRLIDATLYVTFEPCVMCAGAMIHSRIGRVVFGVRNNKHGAAGSLVNVLNYPGMNHRVEITEGILADECTALLCDFYRMPRQVFNARKKAQSSISPDGSSGGSSGSETPGTSESATPESSGGSSGGSAKNTITKTLKLRIVRPYNSAEVEKIVADEKNNREKIALEENKDKVKEACSRHLKVAAYCTTRVERNACLFCKARRLDDKFYQKLRGQFPDAVFWQEIGEIFRQLQKQAAEIYNQSLVELYYEILIKGKGIANAGSVEHYLSDVCYTRAAKLFKNAAIASGLRNKIKSNFRLKELRNMKSGLPTTKSDNFPIPLVRQKGGQYTGFEISNHDGDFIIKIPFGRWQVKKEIDKHRPWEKFDFEQVRKSPKPISLLLSTQRRKRNKGWSKDEGTEAEIRKVMSGDYQTSYIEVKRGSKIGEKSAWMLNLSIDVPKIDKGVDPSIIGGIDVGVKSPLVCAINNAFCRYSISDNDLFHFNKKMFARRRILLKKSRHKRAGHGAKNKLKPISILTEKSKRFRKKLIERWACEIADFFIKNKVGTVQMENLESMKRKEDSYFNIRLRGFWPYAEMQNKIEFKLKQYGIEIRKVAPNNTSKTCSKCGHLNNYFNFEYRKKNKFPHFKCEKCNFKENADYNAALNISNPKLKSTKEEP

SEQ ID NO: 2036 - protein, 726 aa, synthetic construct; identical to SEQ ID NO: 684

SEQ ID NO: 2037 - protein, 726 aa, synthetic construct; identical to SEQ ID NO: 684

SEQ ID NO: 2038 - protein, 726 aa, synthetic construct; identical to SEQ ID NO: 684

SEQ ID NO: 2039 - protein, 726 aa, synthetic construct; identical to SEQ ID NO: 684

SEQ ID NO: 2040 - protein, 726 aa, synthetic construct
SEVEFSHEYWMRHALTLAKRARDEREVPVGAVLVLNNRVIGEGWNRAIGLHDPTAHAEIMALRQGGLVMQNYRLSDATLYVTFEPCVMCAGAMIHSRIGRVVFGVRNSKRGAAGSLMNVLNYPGMNHCVEITEGILVDECAALLCDFYRMPRQVLSAQKKAQSSVSSGGSSGGSCGSETPGASGSVTPKSSVGSSAGSTKNTLTKTLKLRIVRPYNSAEVEKIVADEKNNRERIALEKNKDKVKEACSKHLKVAAYCTTQVERNACLFCKARKLDDKFYQKLRGQFPDAVFWQETGEIFRQLQRQAAEIYNQSLIELYYEIFIKGKGFANASSVEHYLSDVCYTRAAELFKNAAIASGLRGKVKGNFRLKELKNMKSGLPTTKSDNFPIPLVKQKGGQYTGFEISSHNDDFIIKIPFGKWQAKKEIDKYRPWEKFDFEQVRKSPKPISLLLSTQRRKKNKGWSKDEGTEAEIRKVMNGDYQTSYIEVKRGSKIGEKSAWMLNLSIDVPKIDKGVDPSIIGGIDVGVKSPLVCAINNSSSRYSICDNDLFRFNKKMFARRRILLKKNRHKRAGHGAKNKLKPITILTKKSERFRKKLIERWVCEVADFFIKNKVGTVQMENLESMKRKEDSYFNIRLRGFWPYAEMQNKIEFKLKQYGIEIRKVAPNNTSKTCSKCGHLNNYFSFEYRKKNKFPHFKCEKCNFKENADYNAALNISNPKLKSTKEEP

SEQ ID NO: 2041 - protein, 726 aa, synthetic construct
SEDEFSHEYWMRHALTLAKRARDEREVPVGAVLVLNNRVIGEGWNRAIGLHDPTAHAEIMALRQGGLVMQNYRLTEATLYVTFEPCVMCAGAMIHSRIGRVVFGVRNSKRGAAGSLMNVLNYPGMNHCVEITEGILVDECAALLCDFYRMPRQVLNAQKKAQSSISSGGSSGGSSGSETPGTSECPTPESSGGSSGGSAKNTITKTLKLRIVRPYNSAEVEKIVAEEKDNREKIALERNKDKVKEACSKHLKVASYCTTQVERNACLFCKARKLDDKFYQKLRGQFPDAVFWQELGEIFRQLQKQAAEIYNQSLIELYYEIFIKGRGFANASSVEHYLSDVCYTRAAELFKNAAIASGLRGKVKGNFRLKELKSMKSGLPTTKSDNFPIPLVKQKGGQYTGFEISSHNDDFIIKIPFGRWQVKKEIDKYRPWEKFDFEQVRKSPKPISLLLSTQRRRRNKGWGKDEGTEAEIRKVMNGDYQTSYIEVKRGSKTGEKSAWMLNLSIDVPKIDKGVDPSIIGGIDVGVKSPLVCAINNAFSRYSISDNDLFHFNKKMFARRRILLKKNRRRRAGHGAKNKLKPITILTEKSVRFRKKLIERWACEIADFFIKNKVGTVQMENLESMKRKEDSYFNIRLRGFWPYAEMQNKIEFKLKQYGIEIRRVAPNNTSRTCSKCGHLNNYFNFEYRRKYKFPHFKCEKCNFKEDADYNAALNISNPKLKSTKEEP

SEQ ID NO: 2042 - protein, 725 aa, synthetic construct
SEVEFSHEYWMRHALTLAKRARDEREVPVGAVLVLNNRVIGEGWNRAIGLHDPTAHAEIMALRQGGLVMQNYRLSDATLYVTFEPCVMCAGAMIHSRIGRVVFGVRNSKRGAAGSLMNVLNYPGMNHCVEITEGILVDECAALLCDFYRMPRQVLSAQKKAQSSVSSGGSSGGSSGSETPGASGSVTPKSSVGGSAGSTKNTVTKTLKLRIVRPYNSAEVEKIVADEKNNREIALEKNKDKVKEACSKHLKVASYCTTQVERNACPFCKARKLDDKFYQKLRGQFPDAVFWQELGEILRQLQKQAAEIYNQSLIELYYEIFIKGRGFANASSVEHYLSDVCYTRAAELFKNAAIASGLRGKVKSNFRLKELKNMKSGLPTTKSDNFPIPLVKQKGGQYTGFEISSHNDDFIIKIPFGRWQVKKEIDKYRPWEKFDFEQVRKSPKPISLLLSTQRRKKNKGWSKDEGTEAEIRRVMNGDYQTSYIEVKRGSKIGEKSAWMLNLSIDVPKIDRGVDPSIIGGIDVGVKSPLVCAVNNSFSRYSICDNDLFRFNKKMFARRRILLKKNRHKRAGHGTKNKLKPITILTEKSGRFRKKLIERWACEIANFFVKNKVGTVQMEDLESMKRKEDSYFSIRLRGFWPYAEMQNKIEFKLKQYGIEIRKVAPNNTSKTCSKCGHLNNYFNFEYRKKNKFPHFKCEKCNFKEDADYNAALNISNPKLRSTKEEP

SEQ ID NO: 2043 - protein, 726 aa, synthetic construct
SEVEFSHEYWMRHALTLAKRARDEREVPVGAVLVLDNRVIGEGWNRAIGLHDPTAHAEIMALRQGGLVMQNYRLIDATLYVTFEPCVMCAGAMVHSRIGRVVFGVRNNKRGAAGSLMNVLDYPGMDHRVEITEGILADECAALLCDFYRMPRQVFNAQRKAQSSINSGGSSGGSSGSETPGTSESATPESSGGSSGGSAKNTITKTLQLRIVRPYNSAEVEKIVADEKNNREKIALEKNKDKVKEACSKHLKVAAYCTTQVERNACLFCKARKLDDKFYQELRGQFPDAVFWQEIGEIFRQLQKQAAEIYNQSLIELYYEIFIKGKGFANASSAEHYLSDVCYTRAAELFKNAAIASGLRGKVKSNFRLKELKNMKSGLPTTKSDNFPIPLVRQKGGKYTGFEISSHNDDFIIKIPFGRWQVKKEIDKYRPWEKFDFEQVRKSPKPISLLLSTQRRKRNKGWSKDEGTEAEIRKVMNGDYQTSYIEVKRGSKIGEKSAWMLNLSIDVPKIDKGVDPSIIGGIDVGVKSPLVCAINNAFSRYSISDNDLFHFNKKMFARRRILLKKNRHKRAGHGAKNKLKPISILTEKSKRFRKKLIERWACEIADFFIKNKVGTVQMENLESMKRKEDSYFNIRLRGFWPYAEMQNKIEFKLKQYGIEIRKVAPNNTSKTCSKCGHLNNYFNFEYRKMNKFPHFKCEKCNFKENADYNAALNISNPKLKSTKEEP

SEQ ID NO: 2044 - protein, 726 aa, synthetic construct
SEVEFSHEYWMRHALTLAKRARDEREVPVGAVLVLNNRVIGEGWNRAIGLHDPTAHAEIMALRQGGLVMQNYRLIDATLYVTFEPCVMCAGAMIHSRIGRVVFGVRNNKHGAAGSLVNVLNYPGMNHRVEITEGILADECAALLCDFYRMPRQVFNARKKAQSSINPGGSSGGSSGSETPGTSESATPESSGGSSGGSAKNTITKTLKLRIVRPYNSAEVEKIVADEKNNREKIALEKNKDKVREACSKHLRVAAYCTTLVERNACLFCKARRLDDKFYQKLRGQFPDAVFWQEIGEIFRQLQKQAAEIYNQSLVELYYEILIKGKGIANASSVEHYLSDVCYTRAAELFKNAAIASGLRNKIKSNFRLKELRNMKSGLPTTKSDNFPIPLVKQKGGQYTGFEISSHNDDFIIKIPFGRWQVKKEIDKYRPWEKFDFEQVRKSPRPISLLLSTQRRKRNKGWGKDEGTEAEIRKVMNGDYQTSYIEVKRGSKIGEKSAWMLNLSIDVPKIDKGVDPSVIGGIDVGVKSPLVCAINNAFSRHSISDNDLFHFNKKMFARRRILLKKNGRKRAGHGAKNKLKPITILTEKSKRFRKKLIERWACEIAGFFIKNKVGTVQMENLESMKRREDSYFNIRLRGFWPYAEMQNKIEFKLKQYGIEIRKVAPNNTSKTCSKCGHLNNYFNFEYRKKNKFPHFKCEKCSFKENADYNAALNISNPKLKSTKEEP

SEQ ID NO: 2045 - protein, 726 aa, synthetic construct
SEVEFSHEYWMRHALTLAKRARDEREVPVGAVLVLNNRVIGEGWNRAIGLHDPTAHAEIMALRQGGLVMQNYRLVDATLYVTFEPCVLCAGAMVHSRIGRVVFGVRNSKRGAAGSLMNVLNYPGMNHRVEITEGILADECAALLCDFYRMPRQVFNAQKKAQSSISSGGSSGGSSGSETPGASESVTPKSSVGSSASSTKNTITKTLKLRIVRPYNSAEVEKIVADEKDNREKIALEKNKDKVKEACSKHLKVAAYCTTQVERNACLFCKARKLDDKFYQKLRGQFPDAVFWQEISEIFRQLQKQAAEIYNQSLIELYYEIFIKGKGFANASSVEHYLSDVCYTRAAELFKNAAIASGLRGKVKSNFRLKELKNMKSGLPTTKSDNFPIPLVKQKGGQYTGFEISSHNDDFIIKIPFGRWQVKKEIDKYRPWEKFDFEQVRKSPKPISLLLSTRRRKRNKGWSKDEGTEAEIRKVMNGDYQTSYIEVKRGSKIGEKSAWMLNLSIDVPKVDKGVDPSIIGGIDVGVKSPLVCAINNAFSRYSISDNELFHFNKKMFARRRILLKKNRHKRTGHGAKNKLKPISVLTEKSGRFRKKLIERWACEIADFFIKNKVGTVQMENLGSMKRKEDSYFNIRLRGFWPYAEMQNKIEFKLKQYGIEIRKVAPDNTSKTCSKCGHLNNYFNFEYRKRNKFPHFKCEKCNFKEDADYNAALNISNPKLKNTKEEP

SEQ ID NO: 2046 - protein, 726 aa, synthetic construct
SEVEFSHEYWMRHALILAKRARDEREVPVGAVLVLNNRVIGVGWNRAVGLHDPTAHAEIMALRQGGLVMQNNRLIEATLYVTFEPCIMCAGAMIHSRIGRVVFGVRNSKRGAAGSLMNVLNYPGMNHRVEITEGILADECAALLCDYYRMPRQVFNARKKAQSSINSGGSSDGGSGSETPGTCESVTPESSGGSSGGSAKSTITKTLKLRIVRPYNSAEVEKIVADEKNNRERIALEKNKDKVKEACSKHLRVAAYCTTQVERNACLFCKARKLDDKFYQKLRGQFPDAVFWQETGEIFRQLQRQAAEIYNQSLIELYYEIFIKGKGFANASSVEHYLSDVCYTRAAELFKNAAIASGLRGKVKGNFRLKELKNMKSGLPTTKSDNFPIPLVKQKGGQYTGFEISSHNDDFIIKIPFGRWQAKKEIDKYRPWEKFDFEQVRKSPKPISLLLSTQRRKRNKGWSKDEGTEAEIRKVVNGDYQTSYIEVKRGSKIGEKSAWMLNLSIDVPKIDKGVDPSIIGGIDVGVKSPLVCAINNAFSRYSISDNDLFHFNKKMFARRRILLKKNRHKRAGHGAKNKLKPISILTEKSKRFRKKLIERWACEIADFFIKNKVGTVQMENLESMRRKEDSYFNIRLRGFWPYAEMQNKIEFKLKQYGIEIRKVAPNNTSKTCSKCGHLNNYFNFEYRRKNKFPHFKCERCNFKEDADYNAALNISNPKLKSTKEEP

SEQ ID NO: 2047 - protein, 726 aa, synthetic construct
SEVEFSHEYWMRHALTLAKRARDEREVPVGAILVLNNRVIGEGWNRAIGLHDPTAHAEIMALRQGGLVMQNYRLIDATLYVTFEPCVMCAGAMIHSRIGRVVFGVRNSKHGAAGSLVNVLNYPGMNHRVEITEGILADECAALLCDFYRMPRQVFGARRKAQSSINPGGSSGGSSSSETPGTSESPTPESPGGSSGGSAKNTITKTLKLRIVRPYNSAEVEKIVADEKNNREKIALEKNKGKVKEACSKHLEVAAYCTTQVERNACLFCKARKLDDKFYQKLRGQFPDAVFWQELGEIFRQLQKQAAEIYNQSLIELYYEIFIKGKGFANASSVEHYLSDVCYTRAAELFKNAAIASGLRGKVKSNFRLKELKNMKSGLPTTKSDNFPIPLVKQKGGQYTGFEISSHNDDFIIKIPFGRWQVRKEIDKYRPWEKFNFEQVRKSPKPISLLLSTQRRKRNKSWSKDEGTEAEIRKVMNGDYRTSYIEVKRGSKIGEKSAWMLSLSIDVPKIDKGVDPSIIGGIDVGVKSPLVCAINNAFNRYSISDNNLFHFNKKMFARRRILLKKNRHKRAGHGAKNKLKPISILTEKSERFRKKLIERWACEIADFFIRNKVGTVQMENLEGMRRKEDSYFNIRLRGFWPYAEMQNKIEFKLKQYGIEVRKVAPNNTSKTCSKCGHLNNYFNFEYRKKNKFPHFKCEKCNFKENADYNAALNISNPKLKSTKEEP

SEQ ID NO: 2048 - protein, 726 aa, synthetic construct
SEVEFSHEYWMRHALTLAKRARDGREVPVGAVLVLNNRVIGEGWNRAIGLNDPTAHAEIMALRQGGLVMQNHRLIDATLYVTFEPCVMCAGAMVHSRIGRVVFGVRNSKRGAAGSLMNVLDHPGMDHRVEITEGILADECAALLCDFYRMPRQVFNAQKKAQSSISSGGSSGGSSGSETPGTSESATPECPGGSSGGSAKNTITKTLQLRIVRPYNSAEVEKIVADEKNNREKIALEKNKGKVKEACSKHLKVASYCTTQVERNACLFCKARKLDDKFYQKLRGQFPDAVFWQELGEIFRQLQKQAAEIYNQSLIELYYEIFIKGRGFANASSVEHYLSDVCYTRAAELFKNAAIASGLRGKVKGNFRLKELKNMKSGLPTTKSDNFPIPLVRQKGGQYTGFEISSHNDDFIIKIPFGRWQVKKEIDKYRPWEKFDFEQVRKSPKPISLLLSTQRRKRNKGWGKDEGTEAEIRKVMNGDYQTSYIEVKRGSKIGEKSAWMLNLSIDVPKIDKGVDPSIIGGIDVGVKSPLVCAINNAFSRYSISDNDLFHFNKKMFARRRILLKKNGHKRAGHGAKNKLKPITIMTEKSKRFRRKLIERWACEIADFFIKNKVGTVQMENLESMKRKEDSYFNIRLRGFWPYAEMQNKIEFKLKQYGIEIRKVAPNNTSKTCSKCGHLNNYFNFEYRKKNKFPHFKCEKCNFKENADYNAALNISNPELKSTKEEP

SEQ ID NO: 2049 - protein, 726 aa, synthetic construct
SEVEFSHEYWMRHALTLAKRARDEREVPVGAILVLDNRVIGEGWNRAIGLHDPTAHAEILALRQGGLVMQNYRLIDATLYVTFEPCVMCAGAMIHSRIGRVVFGVRNSKHGAAGSLVNVLNYPGMNHRVEITEGILADECAALLCDFYRMPRQVFGARRKAQSSINPGGSSGGSSSSETPGTSESPTPESPGGSSGGSAKNTITKSLKLRIVRPYNSAEVEKIVADEKNNREKVALEKSKGKVKEACSTHLKVATYCTTQVERNACLFCKARKLDDKFYQKLRGQFPDAVFWQEIGEIFRQLQKQAAEIYNQSLIELYYEIFIKGKGFANASSVEHYLSDVCYTRAAELFKNAAIASGLRGKVKSNFRLKELKNMKSGLPTTKSDNFPIPLVKQKGGQYTGFEISSHNDDFIIKIPFGRWQVKKEIDKYRPWEKFDFEQVRKSPKPISLLLSTQRRKRNKGWSQDEGTEAEIRKVMNGDYQTSYIEVKRGSKTGEKSAWMLNLSIDVPKIDKGVDPSIIGGIDVGVKSPLVCAINNAFSRYSISDNDLFHFNKKMFARRRILLRKNGHKRAGHGAKNKLKPITIMTEKSKRFRKKLIERWACEIADFFIKNKVGTVQMENLESMKRKEDSYFNIRLRGFWPYAEMQNKIEFKLKQYGIEIRKVAPNNTSKTCSKCGHLNNYFSFEYRKKNKFPHFKCEKCNFKENADYNAALNISNPKLTSTKEEP

SEQ ID NO: 2050 - protein, 726 aa, synthetic construct
SEVEFSHEYWMRHALTLAKRARDEREVPVGAVLVLNNRVIGEGWNRAIGLHDPTAHAEIMALRQGGLVMQNYRLTDATLYVTFEPCVMCAGAMIHSRIGRVVFGVRNSKHGAAGSLVNVLNYPGMNHRVEITEGILADECAALLCDFYRMPRQVFNARKKARSNINSGGSSGGSSGSEMPGTSESATPESSGGSSGGSAKNTITKTLKLRIVRPYNSAEVEKIVADEKNNREKIALEKNKDKVKEACSEHLKVAAYCTTQVERNACLFCKARKLDDKFYQKLRGQFPDAVFWQEVSEIFRQLQKQAAVIYNQSLIELYYEIFIKGKGFANASSVEHYLSDVCYTRAAELFRNAAIASGLRGKVKSNFRLKELKNMKSGLPTTKSDNFPIPLVKQKGGQYTGFEISSHNDDLIIKIPFGRWQVKKEIDKYRPWEKFDFEQVRKSPKPISLLLSTQRRKRNKGWSKDEGTEAEIRKVMNGDYQTSYIEVKRGSKIGEKSAWMLNLSIDVPKIDKGVDPSIIGGIDVGVKSPLVCAVNNAFSRYSISDNDLFRFNKKMFARRRILLKKNRHQRAGHGAKNKLKPITILTEKSGRFRKKLIERWACEIADFFIKNKVGTVQMENLESMKRKEDSYFNIRLRGFWPYAEMQNKIEFKLKQYGIKIRKVAPNNTSRTCSKCGHLNNYFSFEYRKKNKFPHFKCEKCNFKENADYNAALNISNPKLMSTKEEP

SEQ ID NO: 2051 - protein, 726 aa, synthetic construct
SEVEFSHEYWMRHALTLAKRARDEREVPVGAVLVLNNRVIGEGWNRAIGLHDPTAHAEIMALRQGGLAMQNYRLVDATLYVTFEPCVLCAGAMVHSRIGRVVFGVRNSKRGAAGSLMNVLNHPGMNHRVEITGGILADECAALLCDFYRMPRQVFNAQKKARSNINSGGSSGGSSGSETLGTSESATPESSGGSSGGSAKNTITKTLQLRIVRPYNSAEVEKIVADEKNNREKIALEKNKDKVKEACSKHLKVASYCTTQVERNACPFCKARKLDDKFYQKLRGQFPDAVFWQELGEILRQLQKQAAEIYNQSLIELYYEIFIKGRGFANASSVEHYLSDVCYTRAAELFKNAAIASGLRGKVKSNFRLKELKNMKSGLPTTKSDNFPIPLVKQKGGQYTGFEISSHNDDFIIKIPFGRWQVKKEIDKYRPWEKFDFEQVRKSPKPITLLLSTQRRKRNKGWSKDEGTEAEIRKVMNGDYQTSYIEVKRGSKTGEKSAWMLNLSIDVPKIDKGVDPSIIGGIDVGVKSPLVCAINNAFSRYSISDNDLFRFNKKMFARRRILLRRNRHKRAGHGTKNKLKPITILTEKSGRFRKKLIERWACEIADFFIKNKVGTVQMENLESMKRREDSYFNIRLRGFWPYAEMQNKIEYKLKQYGIETRKVAPNNTSKTCSRCGHLNNYFSFEYRRKNKFPHFKCEKCNFKENADYNAALNISNPKLKSTKEEP

SEQ ID NO: 2052 - protein, 726 aa, synthetic construct; identical to SEQ ID NO: 684

SEQ ID NO: 2053 - protein, 726 aa, synthetic construct; identical to SEQ ID NO: 684

SEQ ID NO: 2054 - protein, 726 aa, synthetic construct
SEVVFSHEYWMRHALSLAKRARDEREVPVGAVLVLNNRIIGEGWNRAIGLHDPTAHAEIMALRQGGLVMQNYRLTDATLYVTFEPCIMCAGAMVHSRIGRVVFGVRNSKRGAAGSLMNVLNYPGVNHCVEITEGILVDECAALLCDFYRMPRQVLNAQKKAQSSISSGGSSGGCSGSEMPGASESVTPKSSGGSSAGSTKNTITKTLKLRIVRPYNSAEVEKIVADEKNNRERIALEKNKDKVKEACSKHLMVASYCTTQVERSACLFCKARELDDKFYQKLRGQFPDAVFWQELGEILRQLQKQAAEIYNQSLIELYYKIFIKGRGFANASSVEHYLSDVCYTRAADLFKNAAIASGLRGKVKGNFRLKELKNMKSGLPTTKSDNFPIPLVKQKGGQYTGFEISGHNDDFIIKIPFGRWQVKKEIDKYRPWEKFDFEQVRKSPKPISLLLSTQRRKRNKGWSKDVGTEAEIRKVMNGDYQTSYIEVKRGSKIGEKSAWMLSLSIDVPKIDKGVDPSIIGGIDVGVKSPLVCAINNAFSRYSISDNDLFRFNKKVFARRRILLKKNRHKRAGHGTKNKLKPITILTEKSERFRKKLIERWACEIANFFTKNKVGTVQMENLESMKRKEDSYFNIRLRGFWPYAEMQSKIEFKLKQYGIEIRKVAPNNTSKTCSKCGHLNNYFNFEYRKKNKFPHFKCEKCNFKENADYNAALNISNPKLKSTKEEP

SEQ ID NO: 2055 - protein, 726 aa, synthetic construct
SEVEFSHEYWMRRALTLAKRARDEREVPVGAVLVLNNRVIGVGWNRAVGLHDPTAHAEIMALRQGGLVMQNYRLIEATLYVTFEPCIMCAGAMIHSRIGRVVFGVRNSKRGAAGSLMNVLNYPGMNHRVEITEGILADECAALLCDYYRMPRQVFNAQKRAQSSINSGGSSGGSSGSETPGTSESATPESSGGSSGSSAKNTITKTLKLRIVRPYNSAEVEKIVADEKNNREKIALEKNKDKVKEACSKHLKVAAYCTTQVERNACLFCKARKLDDKFYQKLRGQFPDAVFWQEIGEVFRQLQKQAAEIYNQSLIELYYEIFIKGKGFANASSVEHYLSGVCYTRAAELFKNAAIASGLRGKVKSNFRLKELKNMKSGLPTTKSDNFPIPLVKQKGGQYTGFEVSSHNDDFIIKIPFGRWQVKKEIDKYRPWEKFDFEQVRKSPKPISLLLSTQRRKRNKGWSKDEGTEAEIRKVMNGDYQTSYIEVKRGSKIGEKSAWMLNLSIDVPKIDKGVDPSIIGGIDVGVKSPLVCAIHNAFSRYSISDNDLFRFNKKVFARRRILLKKNRHKRAGHGAKNKLKPISILTGKSERFRKKLIERWACEIADFFTKNKVGTVQMENLESMKRKEDSYFNIRLRGFWPYAEMQNKIEFKLKQYGIEIRKVAPNNTSKTCSKCGHLNNYFNFEYRKKNKFPHFKCEKCNFKENADYNAALNISNPKLKSTKEEP

SEQ ID NO: 2056 - protein, 726 aa, synthetic construct
SEVEFSHEYWMRRALTLAKRARDEREVPVGAVLVLNNRVIGVGWNRAVGLHDPTAHAEIMALRQGGLVMQNYRLIEATLYVTFEPCIMCAGAMIHSRIGRVVFGVRNSKRGAAGSLMNVLNYPGMNHRVEITEGILADECAALLCDYYRMPRQVFNARKKAQSGINSGGSSDGGSGSETPGTSESATPESSGGSSGGSAKNTITKTLKLRIVRPYNSAEVEEIVADEKNNREKIALEKNKDKVKEACSEHLKVAAYCTTQVERSACLFCKARKLDDKFYQKLRGQFPDAVFWQELGEIFRQLQKQAAEIYNQSLIELYYEIFIKGKGFANASNVEHYLSDVCYTRAAELFKNAAIASGLRGKVKSNFRLKELKNMKSGLPTTKSDNFPIPLVKQKGGQYTGFEISSHNDDFIIKIPFGRWQVRKEIDKYRPWEKFDFEQVRKSPKPISLLLSTQRRKRNKGWSKDEGTEAEIKKVMNGDYQTSYIEVKRGSKIGEKSAWMLNLSIDVPKIDKGVDPSITGGIDVGVKSPLVCAINNALSRYSISDNDLFHFNKKMFARRRILLKKNRHKRAGHGAKNKLKPISILTEKSERFRKKLIERWACEIADFFIKNKVGTVQMENLESMKRREDSYFSTRLRGFWPYAKMQNKIEFKLKQYGIEIRKVAPNNTSKTCSKCGHLNHYFNFEYRKKNKFPHFKCEKCNFKENADYNAALNISNPKLKSTKGEP

SEQ ID NO: 2057 - protein, 726 aa, synthetic construct
SEVEFSHEHWMRHALTLAKRARDEREVPVGAVLVLNNRVIGEGWNRAIGLHDPTAHAEIMALRQGGLVMQNYRLTDATLYVTFEPCVMCAGAMVHSRIGRVVFGVRNSKHGAAGSLVNVLNYPGMNHRVEITEGILADECAALLCDFYRMPRQVFNAQKRAQSTINSGGSSGGSSGSEAPGTNESPTPESSGGSPGGSAKSTITKTLKLRIVRPYNSAEVEKIVADEKNNREKIALEKNKDKVKEACSKHLKVAAYCTTQVERDACLFCRARKLDDKFYQRLRGQFPDAVFWQEIGEIFRQLQKQAAEIYNQSLIELYYEIFIKGKGFANASSVEHYLSDVCYTRAAELFKNAAIASGLRGKVKSNFRLKELKNMKSGLPTTKSDNFPIPLVKQKGGQYAGFEISSHNDDFIIKIPFGRWQVKKEIDKYRPWEKFDFEQVRKSPKPISLLLSTRRRKRNKGWSKDEGTEAEIRKVMNGDYQTSYIEVKRGSKIGEKSAWMLNLSIDVPKIDKGVDPSIIGGIDVGVKSPLVCAINSAFSRYSISDNDLFRFNKKVFARRRILLKKNRHKRAGHGTKNKLKPIAILTEKSGRFRKKLIERWACEIANFFIKNKVGTVQMENLESMKRKEDSYFNIRLRGFWPYAEMQNKIEFKLKQYGIEVRKVAPNNTSKTCSKCGHLNYYFNFEYRKKNKFPHFKCEKCNFKEDADYNAALNISSPKLKSTKEEP

SEQ ID NO: 2058 - protein, 726 aa, synthetic construct
SEAEFSHEYWMRHALTLAKRARDEREVPVGAILVLNNRVIGEGWNRAIGLHDPTAHAEIMALRQGGLVMQNYRLIDATLYVTFEPCVMCAGAMIHSRIGRVVFGVRNNKHGAAGSLVNVLNYPGMNHRVEITEGILADECAALLCDFFRMPRQVFNARKKAQSSINPGGSSGGSSGSETPGTSESATPESSGGSSGSSAKNTITKTLKLRIVRPYNSAEVEKIVADEKDNREKIALERNKGKVKEACSKHLKMAAYCTTQVERNACLFCKARKLDDKFYQKLRGQFPDAVFWQEIGEIFRQLQKQAAEIYNQSLVELYYEILIKGKGIANASSVEHYLSDVCYTRAAELFKNAAIASGLRNKIKSNFRLKELRNMKSGLPTTKSDNFPIPLVRQKGGQYTGFEISNHDGDFIIKIPFGRWQVKKEINKHRPWEKFDFEQVRRSPKPISLLLSTQRRKRNKGWSKDEGTEAEIRKVMNGDYQTSYIEVKRGSKIGEKSAWMLNLSIDVPKIDKGVDPSIIGGIDVGVKSPLVCAINNALSRYSISDNDLFHFNKKMFARRRILLRKNRHKRAGHGAKNKLKPITIMTERSKRFRKKLIERWACEIADFFIKNKVGTVQMENLESMKRREDSYFNIRLRGFWPYAEMQNKIEFKLKQYGIVVRKVAPNNTSKTCSKCGHLNNYFNFEYRKKNKFPHFKCEKCNFKEDADYNAALNISNPKLKSTKGEP

SEQ ID NO: 2059 - protein, 726 aa, synthetic construct
SEVEFSHEYWMRHALTLAKRARDEREVPVGAVLVLNNRVIGEGWNRAIGLHDPTAHAEIMALRQGGLVMRNYRLIEATLYVTFEPCIMCAGAMIHSRIGRVVFGVRNSKRGAAGSLMNVLDYPGMGHRVEITEGILADECAALLCDFYCMPRQVFNAQKRAQSSINSGGSSGGSCGSDTPGTSESATPESSGGGSSGSAKNTITKTLQLRIVRPYNSAEVEKIVADEKNNREKIALEKNKDKVREACSKHLKVASYCTTQVEGNACPFCKARKLDDKFYQKLRGQFPDAVFWQELGEILRQLQKQAAEIYNQSLIELYYEIFIKGKGIASASRVGHYLSDVCYTRAAELFKNAAIASGLRSKIKSNFRLKELKNMKSGLPTTKSDNFPIPLVKQKGGQYTGFEISSHNDDFIIKIPFGRWQMKKEIDRYRPWEKFDFEQVRKSPKPISLLLSTQRRKRNKGWSKDEGTEAEIRKVMNGDYQTSYIEVKRGSKIGEKSAWMLNLSIDVPKVDKGVDPSIIGGIDVGVKSPLVCAINNAFSRYSISDNDLFHFNKKMFARRRILLKKGKHKRAGHGAKNKLKPITILTEKSGRFRKKLIERWACEIADFFIKNKVGTVQMENLESMKRKEDSYFNIRLRGFWPYAEMQNKIEFKLKQYGIEIRKVAPNNTSKTCSKCGHLNHYFNFEYRKKNKFPHFKCEKCNFKENADYNAALNISNPRLKSTREEP

SEQ ID NO: 2060 - protein, 726 aa, synthetic construct
GEDEFSHEYWMRHALTLAKRARDEREVPVGAVLVLNNRVIGEGWNRAIGLHDPTAHAEIMALRQGGLVMQNYRLVDATLYVTFEPCVLCAGAMVHSRIGRVVFGVRNSKRGAAGSLMNVLNYPGMNHRVEITEGILADECAALLCDFYRMPRQVFNAQKKARSNINPGGSSGGSSDSEAPGTSENATPGSSGGSSGGSAKNTITKTLKLRIVRPYNSAEVEKIVADEKNNREKIALEKNKDKVKEACSEHLKVAAYCTTQVERSACLFCKARKLDDKFYQKLRGQFPDAVFWQEIGEIFRQLQKQAAEIYNQSLIELYYEIFIKGKGFANASSVEHYLSDVCYARAAELFKNAAIASGLRGKVKSNFRLKELKNMKSGLPTTKSDNFPIPLVKQKGGQYTGFEISSHNDDFIIKIPFGRWQVKKEIDKYRPWEKFDFEQVRKSPKPISLLLSTQRRKRNKGWSKDEGTEAEIRKVMNGDYQTSYIEVKRGSKIGEKSAWMLNLSIDVPKIDKGVDPSIIGGIDVGVRSPLVCAINNAFSRYSISDNDLFRFNKKMFARRRILLKKNRHRRAGHGAKNKLKPVTILTEKSRRFRKKLIERWACEIANFFIKNKVGTVQMENLESMKRKEDSYFNIRLRGFWPYAEMQNKIEFKLKQYGIKIRKVAPNNTSKTCSKCGHLNNYFSFEYRKKNKFPHFKCEKCNFKENADYNAALNISNPKLKSTKEEP

SEQ ID NO: 2061 - protein, 726 aa, synthetic construct
SEVEFSHEYWMRHALTLAKRARDEREVPVGAVLVLNNRAIGEGWNRAIGLHDPTAHAEIMALRQGGLVMQNYRLVDATLYVTFEPCVLCAGAMIHSRIGRVVFGVRNSKRGAAGSLMNVLNYPGMNHRVEITEGILADECAALLCDFYRMPRQVFNARKKARSNINSGGSSGGSSGSETLGTREGATPESSGGSSAGSTKDTITKTLKLRIVRPYNSAEVEKVVADEKNNREKIAIEKNKDMVKEACSKHLKVASYCTTQVERNACLFCKARKLDDKFYQKLRGQFPDAVFWQELGGIFRQLQKQAAEIYNQSLIELYYEIFIKGRGFANASSVEHYLSDVCYTRAAELFKNAAIASGLRSKVRSNFRLKELKNMKSGLPTTKSDNFPIPLVKQKGGQYTGFEISSHNSDFIIKIPFGRWQVKEEIDKYRPWEKFDFEQVRKSPKPISLLLSTQRRKKNKGWSKDEGTEAEIRRVMNGDYQTSYIEVKRGSKIGEKSAWMLNLSIDVPKIDKGVDPSIIGGIDVGVKSPLVCAINNSSSRYSICDNDLFRFNKKMFARRRILLKKNRHKRAGHGAKNKLKPITILTKKSERFRKKLIERWACEVADFFIRNKVGTVQMENLESMKRKEDSYFNIRLRGFWPYAEMQNRIEFKLKQYGIKIRKVAPNNTSKTCSKCGHLNNYFNFEYRKKNKFPHFKCEKCNFKENADYNAALNISNPKLKSTKEGP

SEQ ID NO: 2062 - protein, 726 aa, synthetic construct
SEVEFSHEYWMRHALTLAKRARDEREVPVGAVLVLNNRVIGEGWNRAIGLHDPTAHAEIMALHQGGLVMQNYRLIDATLYVTFEPCVMCAGAMIHSRIGRVVFGARNSKRGAAGSLMNVLSYPGMNHRVEITEGILADECAALLCDFYRMPRRVFNAQKKAQSSINSGGSSGGGSGSETPGTSESATPESSGGGSGGSAKNTITKTLKLRIVRPYNSAEVEKIVADEKNSREKIALEKNKGKVKEACSKHLKVATYCTTQVERNVCLFCKARKLDDKFYQKLRGQFPDAVFWQEISEIFRQLQKQAAEIYNQSLIELYYEIFIKGKGIANASSVGHYLSDVCYTRAAELFKNAAIASGLRGKIKSNFRLKELRNMKSGLPTTKSDNFPIPLVKQKGGQYTGFEISNHNSDFIIKIPFGRWQAKKEIDKYRPWEKFDFEQVRKSPKPISLLLSTQRRKRNKGWSKDEGTEAEIKKVMNGDYQISYIEVKRGSKIGEKSAWTLNLSVDVPKMEKGVDPSIIGGIDVGVKSPLVCAVNNAFSRYSISDNDLFHFNKKMFARRRILLKKNRHRRAGHGAKNKLRPITILTEKSKRFRRKLIERWACEIADFFIKNKVGTVQMENLESMKRKEDSYFNIRLRGFWPYAEMQNKIEFKLKQYGIEIRKVAPNNTSKTCSKCGHLNNYFNFEYRKKNKFPHFKCEKCNFKENADYNAALNISNPKLKSTKEEP

SEQ ID NO: 2063 - protein, 726 aa, synthetic construct
SEVEFSHEYWMRHALTLARRARDGREVPVGAVLVLNNRVIGEGWNRAIGLHDPTAHAEIMALRQGGLVMQNYRLVDATLYVTFEPCVLCAGAMVHSRIGRVVFGVRNSKRGAAGSLMNVLNYPGMNHRVEITEGILADECAALLCDFYRMPRQVFNARKKARSNINSGGSSGGSSGSETPGTSESPTPESPGGSSGGSAKNTITKTLKLRIVRPYNSAEVEKIVADEKNNREKIALEKNKDKVKEACSKHLKMASYCTTQVERNACLFCKARKLDDKFYQKLRGQFPDAVFWQELGGIFRQLQKQAAEIYNQSLIELYYEIFIKGKGITNASRVEHYLSDVCYTRAAELFKNAAIASGLRSKTKSNFRLKELKNMKSGLPTTRSDNFPIPLVKQKGGPYTGFEISNHNSDFIIKIPFGRWQVKKEIDKYRPWEKFDFEQVRKSPKPISLLLSTQRRKRNKGWGKDEGTEAEIRKVMNGDYQTSYIEVKRGSKIGEKSAWMLNLSIDVPKIDKGVDPSIIGGIDVGVKSPLVCAINNALSRYSISDNDLFHFNKKMFARRRILLRKNRHKRAGHGVRNKLKPITVLTEKSERFRKKLIERWACEIANFFIKNKVGTVQMENLESMKRREDSYFNIRLRGFWPYAEMQSKIEFKLKQYGIKIRKVAPNNTSKTCSRCGHLNNYFNFEYRKKSKFPHFKCEKCNFKEDADYNAALNISNPKLKSTKEEP

SEQ ID NO: 2064 - protein, 726 aa, synthetic construct
SEVEFSHEYWMRHALTLAKRARDGREVPVGAVLVLNNRVIGEGWNRAIGLHDPTAHAEIMALRQGGLVLQNYRLIDATLYVTFEPCVMCAGAMIHSRIGRVVFGVRNNKHGAAGSLVNVLNYPGMNHRVEITEGILADECAALLCDFYRMPRQVFNARKKTQSSINPGGSSGGSSGSETPGTSESATPESSGGSSGSSAKNTITKTLQLRIVRPYNSAEVEKIVADEKNNREKIALEKNKGKVKEACSKHLKVASYCTTQVERNACLFCKARKLDDKFYQKLRGQFPDAVFWQELGEIFRQLQKQTAEIYNQSLIELYYEIFIKGKGFANASSVEHYLSDVCYSRAAELFKNAAIASGLRGKVKSNFRLKELKNMKSGLPTTKSDNFPIPLVKQKGGQYTGFEISSHNDDFIIKIPFGRWQVKEEIDKYRPWEKFDFEQVRKNPKPISLLLSTQRRKRNKGWSKDEGTEAVIRKVMNGDYQTSYIEVKRGSKIGEKSAWMLNLSIDVPKIDKGVDPSIIGGIDVGVKSPLVCAINNAFSRYGISDNDLFRFNKKVFARRRILLKKNRYKRAGHGTKNKLKPITILTEKSGRFRKKLIERWACEIADFFIKNKVGTVQMENLESMKRKEDSYFNIRLRGFWPYAEMQNKIEFKLKQYGIEIRKVAPNNTSKTCSKCGHLNNYFNFEYRKKNKFPHFKCEKCNFKENADYNAALNISNPKLKSTKEEP

SEQ ID NO: 2065 - protein, 726 aa, synthetic construct
SEVEFSHEYWMRHALTLAKRARDEREVPVGAVLVLNNRVIGEGWNRAIGLHDPTAHAEIMALRQGGLVMQNYRLVDATLYVTFEPCVLCAGAMVHSRIGRVVFGVRNSKRGAAGSLMNVLNYPGMNHRVEITEGILADECAALLCDFYRMPRQVLNAQKKARSNINTGGLSGGSSGSETPGASESVTPKSSGGSSTGSTKNTITKTLKLRIVRPYNSAEVEKIVADEKNSREKIALEKNKDKVKEACSKHLKVAAYCTTQVERNACLFCRARRLDDKFYQKLRGQFPDAVFWQEIGEIFRQLQKQAAEIYNQSLVELYYEIFIKGKGIANASSVEHYLSDVCYTRAAELFKNAAIASGLRNKVKSNFRLKELRNMKSGLPTTKSDNFPIPLVRQKGGQYTGFEISNHNSDFIIKIPFGRWQVKKEIDKYRPWEKFDFAQVRKSPKPISLLLSTQRRKRNKGWSNDEGTEAEIRKVMNGDYQTSYIEVKRGSKIGEKSAWMLNLSIDVPKIDKGVDPSIIGGIDVGVKSPLVCAINNSSSRYSICDNDLFRFNKKMFARRRILLKKNRHKRAGHGAKNKLKPITILTKKSERFRKKLIERWVCEVADFFIKNKVGTVQMENLESMKRKEDSYFNIRLRGFWPYAEMQNRIELKLKQYGIEIRRVAPNNTSRTCSKCGHLNNYFNFEYRKKSKFPLFKCEKCNFREDADYNAALNISNPKLKGTKEEL

SEQ ID NO: 2066 - protein, 726 aa, synthetic construct
SEVEFSHEYWMRHALTLAKRARDEREVPVGAVLVLNNRVIGEGWNRTTGLHDPTAHAEIMALRQGGLVMRNYRLTDATLYVTFEPCVMCAGAMIHGRIGRVVFGVRNSKRGAAGSLMNVLNYPGMNHCVEITEGILVDECAALLCDFYRMPRQVLNAQKKAQSSISPGGSSGGSSGSETPSASESVTPKSSGGSSGGSAKNTITKTLKLRIVRPYNSAEVEKIVADEKNNREKIALEKNKGKVKEACSKHLEVAAYCTTQVERNACLFCKARKLDDKFYQKLRGQFPDAVFWQELGEIFRQLQKQAAEIYNQSLIELYYEIFIKGKGFANASSVEHYLSDVCYTRAAELFKNAAIASGLRGKVKSNFRLKELKNMKSGLPTTKSDNFPIPLVKQKGGQYTGFEISSHNDDFIIKIPFGRWQVKKEIDKYRPWEKFDFEQVRKSPKPISLLLSTQRRRRNKGWSKDEGTEAEIRRVMNGDYQTSYIEVKRGSKTGEKSAWMLNLSIDVPKIDKGVDPSIIGGIDVGVKSPLVCAINNSSSRYSICDNDLFRFNKKMFARRRILLKKNRHKRAGHGAKNKLKPITILTKKSERFRKKLIERWVCEVADFFIKNKVGTVQMENLESMKRKEDSYFNIRLRGFWPYAEMQNRIELKLKQYGIEIRRVAPNNTSRTCSKCGHLNNYFNFEYRKKNKFPHFKCEKCNFKENADYNAALNISNPKLKSTKEKP

SEQ ID NO: 2067 - protein, 726 aa, synthetic construct
SEVEFSHEYWMRHALTLAKRARDECEVPVGAILVLNNRVIGEGWNRAIGLHDPTAHAEIMALRQGGLVMQNYRLIDATLYVTFEPCVMCAGAMIHSRIGRVVFGVRNSKHGAAGSLMNVLNYPGMNHRVEITEGILADECAALLCDFYRMPHQVFSARKKAQSSINPGGSSGGSSGSKTPGTSESATPESSGGSSGGSAKNSITKTLKLRIVRPYNSAEVEKIVADEKNNREKIALEKNKGKVKEACSKHLKVATYCTTQVERNACLFCKARKLDDKFYQKLRGQFPDAVFWQEIGEIFRQLQKQAAEIYNQSLIELYYEIFIEGKGFANASSVEHYLSDVCYTRAAELFKNAAIASGLRGKVKGNFRLKELKSMKSGLPTTKSDNFPIPLVKQKGGQYTGFEISSHNDDFIIKIPFGRWQVKKEIDKYRPWEKFDFEQVRKSPKPISLLLSTRRRKRNKGWSKDEGTEAEIRKVMNGDYQTSYIEVKRGSKIGEKSAWMLNLSIDVPKIDKGVDPSIIGGIDVGVKSPLVCAINNALSRYSISDNDLFHFNKKMFARRRILLRKNRHKRAGHGAKNKLKPITMMTEKSKRFRKKLIERWACEIADFFIKNKVGTVQMENLESMKRKEDSYFNIRLRGFWPYAEMQDKIEFKLKQYGIVVRKVAPNNTSKTCSKCGHLNHYFSFEYRKKNKFPHFKCEKCNFKEDADYNAALNISNPKLKSTKGEP

SEQ ID NO: 2068 - protein, 726 aa, synthetic construct
SEVEFSHEYWMRHALTLAKRARDEREVPVGAVLVLNNRVIGEGWNRATGQNDPTAHAEIMALRQGGLVMQNHRLIDATLYVTFEPCVMCAGAMIHSRIGRVVIGVRNSRRGAAGSLMNVLNHPGMNHRVEITEGILADECAALLCDFYRMPRQVFNAQEKAQSSTNSGGSSGGSSGSETPGTSESVTPESSGGGSSGSAKNTITKTLQLRIVRPYNSAEVEKIVADEKNNREKIALEKNKDKVREACNKHLKVASYCTTQVERNACPFCKARKLDDKFYQKLRGQFPDAVFWQELGEILRQLQKQAAEIYNQSLIELYYEIFIKGKGFANASSVEHYLSDVCYTRAAELFKNAAIASGLRGKVKSNFRLKELRNMKSGLPTTKSDNFPIPLVRQKGGQYTGFEISNHNDDFIIKIPFGRWQVKKEIDKYRPWEKFDFEQVRKSPKPISLLLSTQRRKRNKGWSKDEGTEAEIRKVMNGDYRTSYIEVKRGSKTGEKSAWVLNLSIDVPKIDKGVDPSIIGGIDVGVKSPLVCAINNAFSRYSISDNDLFRFNKKMFARRRILLKKNRHKRAGHGAKNKLKPISILTGKSERFRKKLIERWACEIANFFIKNKVGTVQMENLESMKGREDSYFNIRLRGFWPYAEMQNKIEFKLKQYGIEIRKVAPNNTSKTCSKCGHLNNYFNFEYRKKNKFPHFKCEKCNFKEDADYNAALNISNPKLKSTKEEP

SEQ ID NO: 2069 - protein, 726 aa, synthetic construct
SEDEFSHEYWMRHALTLAKRARDGREVPVGAVLVLNNRVIGEGWNRAIGLHDPTAHAEIMALRQGGLVMQNYRLIDATLYVTFEPCVMCAGAMVHSRIGRVVFGVRNSKRGAAGSLMNVLDYPGMGHRVEITEGILADECAALLCDFYCMPRQVFNAQKRAQSSINSGGSSGSSSGSETPGTSESVTPKSSGGSSGGSAKNTITKTLKLRIVRPYNSAEVEKIVADEKNNREKIALEKNKGKVKEACSKHLEVAAYCTTQVERNACLFCKARKLDDKFYQKLRGQFPDAVFWQELGEIFRQLQKQAAEIYNQSLIELYYEIFIKGKGFANASSVEHYLSDVCYTRAAELFKNAAIASGLRNKIKSNFRLKELRNMKSGLPTTKSDNFPIPLVRQKGGQYTGFEISNHNGDFIIKIPFGRWQVKKEIDKYRPWEKFDFEQVRKSPKPISLLLSTQRRKRNKGWSKDEGTEAEIRKVMNGDYQTSYIEVKRGSKIGEKSAWMLNLSIDVPKIDKGVDPSIIGGIDVGVKSPLVCAINNAFGRYSISDNDLFHFNKKMFARRRILLKKNRHKRAGHGAKNKLKPITILTEKSKRFRKKLIERWACEIANFFIKNKVGTVQMENLEGMKRKEDSYFNIRLRGFWPYAEMQNKIEFKLKQYGIEIRKVAPNNTSKTCSKCGHLNNYFNFEYRKKNKFPHFKCEKCNFKESADYNAALNISNPKLKSTKEEP

SEQ ID NO: 2070 - protein, 726 aa, synthetic construct
SEVEFSHEYWMRHALTLAKRARDEREVPVGAVLVLNNRVIGEGWNRAIGLHDPTAHAEIMALRQGGLVMQDYRLTDATLYVTFEPCVMCAGAMIHSRIGRVVFGVRNSKRGAAGSLMNVLNYPGMNHCVEITEGILVDECAALLCDFYRMPRQVLNAQKKAQSSINSGGSSGGSSGSETLGTSESATPESSGGSSGGSAKNTITKTLKLRIVRPYNSAEVEKIVADEKNNREKTALEKNKDKVKEACSKHLKVAAYCTTQVERNACLFCKARKLDDKFYQKLRGQFPDAVFWQEVGGIFRQLQKQAAEIYNQSLIELYYEIFIKGKGFANASSVEHYLSDVCYTRAAELFKNAAIASGLRGKVKSNFRLRELKNMKSGLPTTKSDNFPIPLVKQKGGQYTGFEISNHNSDFIIKIPFGRWQVKKEIDKHRPWEKFDFEQVRKSPKPISLLLSTQRRKRNKGWSKDEGTEAEIKKVMNGDYQTSYIEVKRGSKIGEKSAWMLNLSIDVPKIDKGVDPSIIGGIDVGVKSPLVCAINNSSSRYSICDNDLFRFNKKMFARRRILLKKNRHKRAGHGAKNKLKPITILTKKSERFRKKLIERWACEIADFFIKNKVGTVQMENLESMKRKEDSYFNIRLRGFWPYAEMQNKIEFKLKQYGIEIRKVAPNNTSKTCSKCGHLNHYFNFEYRRKNKFPHFKCEKCNFRENADYNAALNISNPKLKSTKGEP

SEQ ID NO: 2071 - protein, 726 aa, synthetic construct
SEVEFSHEYWMRHALTLAKRARDEREVPVGAVLVLNNRVIGEGWNRAIGLHDPTAHAEIMALRQGGLVMQNYRLIDATLYVTFEPCVMCAGAMVHSRIGRVVFGVRNSKRGAAGSLMNVLDYPGMGHRVEITEGILADECAALLCDFYCMPRQVFNAQKRAQSSINSDGSSGGSSGSETPGTSESATPESSGGGSSGSAKNTITKTLQLRIVRPYNSAEVEKIVADEKNNREKIALERNKDKVKEACSKHLKVAAYCTTQVERNACLFCKARKLDDKFYQKLRGQFPDAVFWQEIGEIFRQLQKQAAEIYNQSLVELYYEIFVKGKGIVNASSVEHYLSDVCYTRAAGLFKNAAIASGLRNKIKSNFRLKELKNMKSGLPTTKSDNFPIPLVKQKGGQYTGFEISSHNSDFIIKIPFGRWQVKKEIDKYRPWEKFDFEQVRKSPKPISLLLSTQRRKRNKGWSKDEGTEAEIRKVMNGDYQTSYIEVKRGSKIGEKSAWMLNLSIDVPKIDKGVDPSIIGGIDVGVKSPLVCAINNAFSRYSISDNDLFHFNKKMFARRRILLRKNRHKRAGHGAKNKLKPITIMTEKSKRFRKKLIERWACEIADFFIKNKVGTVQMENLESMKRREDSYFNIRLRGFWPYAEMQNKIEFKLKQYGIEIRKVAPNNTSKTCSRCGHLNNYFNFEYRKRNKFPHFKCEKCNFKENADYNAALNISNPKLKSTKEEP

SEQ ID NO: 2072 - protein, 726 aa, synthetic construct
SEVEFSHEYWMRHALTLAKRARDEREVPVGAILVLNNRVIGEGWNRAIGLHDPTAHAEIMALRQGGLVMQNYRLIDATLYVTFEPCVMCAGAMIHSRVGRVVFGVRNSKHGAAGSLMNVLNYPGMNHRVEITEGILADECAALLCDFYRMPRRVFNARKKAQSSIDPGGPSGGSSCSETPGASESVTPKSSGGSSTGSTKNTITKTLKLRIVRPYNSAEVEKIVADEKNNREKIALEKNKDKVKEACSKHLKVAAYCTTQVERNACLFCKARRLDDKFYQKLRGQFPDAVFWQEIGEIFRQLQKQAAEVYNQSLVELYYEILIKGKGIANASSVEHYLSDVCYTRAAELFKNAAIASGLRNKIKSNFRLKELRNMKSGLPTTKSDNFPIPLVRQKGGQYTGFEISNHDGDFIIKIPFGRWQVKKEINKHRPWEKFDFEQVRKSPKPISLLLSTQRRKRNKGWSKDEGTEAEIRKVMNGDYQTSYIEVKRGSKIGEKSAWMLNLSIDVPKIDKGVDPSIVGGIDVGVKSPLVCAINNAFSRYSISDNDLFHFNKKMFARRRILLRKNRHKRAGHGAKNKLKPISILTEKSERFRKKLIERWACEIADFFIKNKVGTVQMENLESMKRREDSYFNIRLRGFWPYAKMQNKIEFKLKQYGIEIRKVAPNNTSKTCSKCGHLNDYFNFEYRKKNKFPHFKCEKCNFKESADYNAALNISNPKLKSTKEEP

SEQ ID NO: 2073 - protein, 726 aa, synthetic construct
SEVEFSHEYWMRRALTLAKRARDEREVPVGAVLVLNNRVIGVGWNRAVGLHDPTAHAEIMALRQGGLVMQNYRLIEATLYVTFEPCIMCAGAMIHSRIGRVVFGVRNSKRGAAGSLMNVLNYPGMNHRVEITEGILADECAALLCDYYRMPRQVFNARKKAQSSINSGGSSGGSSGSEMPGTSESATPESSGGSSGGSARNTITKTLKLRIVRPYNSAEVEKIVADEKNNREKIALEKNKDKVKEACSEHLKVAAYCTTQVERNACLFCKARKLDDKFYQKLRGQFPDAVFWQELGEILRQLQKQAAEIYNQSLIELYYEIFIKGRGFANASSVEHYLSDVCYTRAAELFKNAAIASGLRGKVKSNFRLKELKNMKSGLPTTKSDNFPIPLVKQKGGQYTGFEISSHNSDFIIKIPFGRWQVKEEIDKYRPWEKFDFEQVRKSPKPISLLLSTQRRKKNKGWSKDEGTEAEIRRVMNGDYQTSYIEVKRGSKIGEKSAWMLNLSIDVPKIDKGVDPSIIGGIDVGVKSPLVCAINNSSSRYSICDNDLFRFNKKMFARRRILLKKNRHKRAGHGAKNKLKPITILTKKSERFRKKLIERWACEIADFFIKNKVGTVQMENLESMKRKEDSYFNIRLRGFWPYAEMQNRIELKLKQYGIEIRRVAPNNTSRTCSKCGHLNNYFNFEYRKKSKFPHFKCEKCNFREDADYNAALNISNPKLKSTKEEP

SEQ ID NO: 2074 - protein, 726 aa, synthetic construct
SEVEFSHEYWMRHALTLAKRARDEREVPVGAVLVLNNRVIGEGWNRAIGLHDPTAHAEIMALHQGGLVMQNYRLIDATLYVTFEPCVMCAGAMIHSRIGRVVFGARNSKRGAAGSLMNVLSYPGMNHRVEITEGILADECAALLCDFYRMPRRVFNAQKKAQSTINSGGSSGGSSGSETPGTSESPTPESSGGSPGGSAKNTITKTLKLRIVRPYNSAEVEKIVADEKNNREKIALEKNKDKVKEACSKHLKVAAYCTTQVERNACLFCKARKLDDKFYQKLRGQFPDAVFWQEIGEIFRQLQKQAAEIYNQSLIELYYEIFIKGKGFANASSVEHYLSDVCYTRAAELFKNAAIASGLRGKVKSNFRLKELKNMKSGLPTTKSDNFPIPLVKQKGGQYTGFEISSHNDDFIIKIPFGRWQVRKEIDKYRPWEKFNFEQVRKSPKPISLLLSTQRRKRNRGWSKDESTEAEIRKVMNGDYQTSYIEVKRGSKIGEKSAWMLNLSIDVPKIDKGVDPSIIGGIDVGVKSPLVCAIDNALSRYSISDNDLFHFNKKMFARRRILLRKNRHKRAGHGAKNKLKPITMMTEKSKRFRKKLIERWACEIADFFIKNKVGTVQMENLESMKRKEDGYFNIRLRGFWPYAEMQNKIEFKLKQYGIVVRKVAPNNTSKTCSKCGHLNNYFNFEYRKKNKFPHFKCEKCNFKEDADYNAALNISNPKLKSTKGEP

SEQ ID NO: 2075 - protein, 726 aa, synthetic construct
SEVEFSHEYWMRHALTLAKRARDGREVPVGAVLVLNNRVIGEGWNRAIGLHDPTAHAEIMALRQGSLVMQNYRLIDATLYVTFEPCAMCAGAMVHSRIGRVVFGVRNSKRGAAGSLVNVLNYPGMDHRVEITGGILADECAALLCDFYRMPRRVFNAQKKAQSSINSGGSSGGSSGSVTPGTSESATPESSGGSFGGSAKNTITKTLQLRIVRPYNSAEVEKIVADEKNSREKIALEKNKDKVKEACGKHLKVASYCTTQVERSACLFCKARKLDDKFYQKLRGQFPDAVFWQELGEIFRQLQKQAAEIYNQSLIELYYEIFIKGRGFANASNVEHYLSDVCYTRAAELFKNAAIASGLRGKVKGNFRPKELKNMKSGLPTTKSDNFPIPLVKQKGGQYTGFEISSHNDDFIIKIPFGRWQVKKEIDKYRPWEKFDFEQVRKSPKPISLLLSTQRRKRNKGWSKDEGTEAEIRKVMNGDYQTSYIEVKRGSKTGEKSAWMLNLSIDVPKIDKGVDPSIIGGIDVGVKSPLVCAINNTFSRYSISDNDLFRFNKKMFARRRILLKKNRHKRAGHGAKNKLKPISILTGKSERFRKKLIERWACEIADFFIKNKVGTVQMENLESMKRKEDSYFNIRLRGFWPYAEMQNKIEFKLKQYGIEIRKVAPNNTSKTCSKCGHLNNYFNFEYRKKNKFPHFKCEKCNFKENADYNAALNISNPKLKSTKEEP

SEQ ID NO: 2076 - protein, 726 aa, synthetic construct
SEVEFSHEYWMRHALTLARRARDEREVPVGAILVLNNRVIGEGWNRAIGLHDPTAHAEIMALRQGGLVMQNYRLIDATLYVTFEPCVMCAGAMIHSRIGRVVFGVRNNKHGAAGSLTNVLNYPGMNHRVEITEGILVDECAALLCDFYRMPRQVFNAQKKAQSTINSGGSSGGSSGSETPGTSESPTPKSSGGSSGGSAKNTITKTLKLRIVRPYNSAEVEKIVADEKNNREKIALEKNKDKVKEACSKHLKVAAYCTTQVERNACLFCKARKLDDKFYQKLRGQFPDAVFWQEIGEIFRQLQKQAAEIYNQSLIELYYEIFIKGKGTANASSVEHYLSDVCYTRAAELFKNAAIASGLRNKIKSNFRLKELKNMKSGLPTTKSDNFPIPLVKQKGGQYTGFEISSHNDDFIIKIPFGRWQVKEEIDKYRPWEKFDFEQVRKSPKPISLLLSTQRRRRNKGWSKDEGTEAEIKKVMNGDYQTSYIEVKRGSKIGEKSAWMLNLSIDVPKIDKGVDPSIIGGIDVGVKSPLVCAINNACSRYSISDNDLFHFNKKMFARRRILLKKNRHKRAGHGTKNKLKPITILTEKSGRFRKKLIERWACEIANFFIKNKVGTVQMENLESMKRKEDSYFNIRLRGFWPYAEMQNKIEFKLKQYGIKIRKVAPNNTSKTCSKCGHLNNYFSFEYRKKNKFPHFKCEKCNFKEDADYNAALNISNPKLKSTKEEP

SEQ ID NO: 2077 - protein, 726 aa, synthetic construct
SEVEFSHEYWMRHALTLAKRARDGREVPVGAVLVLNNRVIGEGWNRAIGLHDPTAHAEIMALRQGGLVMQNYRLIDATLYVTFEPCAMCAGAMVHSRIGRVVFGVRNSKRGAAGSLMNVLTYPGMDHRVEITGGILADECAALLCDFYRMPRQVFNAQKKARSNINSGGSSGGSSGSETLGTSESATPESSGGSSGGSAKNTIAKTLQLRIVRPYNSADVEKIVADEKNNREKAALEKNKDKVKEACSKHLKVATYCTTQVGRNACLFCKARKLDDKFYQKLRGQFPDAVFWQEISGIFRQLQKQAAEIYNQSLIELYYEIFIKGKGFANASSVEHYLSDVCYTRAAELFKNAAIASGLRGKVKSNFRLKELKNMKSGLPTTKSDNFPIPLVKQKGGQYTGFEISNHNSDFIIKIPFGRWQVKKEINKYRPWEKFDFEQVRKSPKPISLLLSTQRRKRNKGWSKDEGTEAEIRKVMNGDYQTSYIEVKRGSRIGEKSAWMLSLSIDVPKIDRGVDPSIIGGIDVGVKSPLVCAINNAFSRYSISDNDLFRFNKKMFARRRILLKKNRHKRAGHGAKNKLKPISILTGKSERFRKKLIERWACEIADFFIKNKVGTVQMENLESMKRKEDSYFNIRLRGFWPYAEMQNKIEFKLKQYGIKIRKVAPNNTSRTCSKCGHLNNYFSFEYRKKNKFPHFKCEKCNFKEDADYNAALNISNPKLEGTKEEL

SEQ ID NO: 2078 - protein, 726 aa, synthetic construct
SEVEFSHEYWMRHALILAKRARDEREVPVGAVLVLNNRVIGVGWNRAVGLHDPTAHAEIMALRQGGLVMQNYRLIGATLYVTFEPCAMCAGAMIHGRIGRVVFGVRNSKRGAAGSLMNVLNHPGMNHRVEIMEGILTDECAALLCDFYRMPHQVLNAQKKAQSSINSGGSSGGSSGSETPGTSGSATPEGSGGSSGGSTKNTITKTLKLRIVRPYNSAEVEKIVADEKNNREKIALEKNKGKVKEACSKHLKVAAYCTTQVERNACLFCKARKLDDKFYQKLRGQFPDAVFWQEISEIFRQLQKQAAEIYNQSLIELYYEIFIKGKGFANASSVEHYLSDVCYTRAAELFKNAAIASGLRGKVKSNFRLKELKNMKSGLPTTKSDNFPIPLVKQKGGQYTGFEISNHNDDFIIKIPFGRWQVKKEIDKYRPWEKFDFEQVRKSPKPISLLLSTQRRKRNKGWSKDEGTEAEIRKVMNGDYQTSYIEVKRGSKIGEKSAWMLNLSIDVPKIDKGVDPRIIGGIDVGVKSPLVCAINNAFSRYSISDNDLFHFNKKMFARRRILLKKNRHRRAGHGAKNKLKPISILTEKSKRFRKKLIERWACEIANFFIKNKVGTVQMENLESMKRKEDSYFNIRLRGLWPYAEMQNKIEFKLKQYGIEIRKVAPNNTSKTCSKCGHLNNYFNFEYRRKNKFPHFKCEKCNFKENADYNAALNISNPKLKSTKEEP

SEQ ID NO: 2079 - protein, 726 aa, synthetic construct
SEVEFSHEYWMRHALTLAKRARDEREVPVGAVLVLNNRVIGEGWNRAIGLHDPTAHAEIMALRQGGLVMQNYRLTDATLYVTFEPCVMCAGAMIHSRIGRVVFGVRNSKRGAAGSLMNVLNYPGMNHCVEITEGILVDECAALLCDFYRMPRQVLNAQKKAQSSISSGGSSGGSSGSETPGASESVTPKSSVGSSAGSTKNTITKTLKLRIVRPYNSAEVEKIVADEKNNREKIALEKSKGKVKEACSKHLEVAAYCTTQVERNACLFCKARKLDDKFYQKLRGQFPDAVFWQELGEIFRQLQKQAAEIYNQSLIELYYEIFVKGKGFANASSVEHYLSDVCYTRAAELFKNAAIASGLRGKVKSNFRLRELKSMRSGLPTTKSDNFPIPLVKQKGGQYTGFEISSHDDDFVIKIPFGRWQVKKEIDKYRPWEKFDFEQVRKSPKPISLLLSTQRRKRNKGWSKDEGTEAEIRKVMNGDYQTSYIEVKRGSKIGEKSAWMLNLSIDVPKIDKGVDPSIIGGIDVGVKSPLVCAINNAFSRYSISDNDLFHFNKKMFARRRILLKKSRHKRAGHGAKNKLKPISILTGKSERFRKKLIERWACEIADFFIKNKVGTVQMENLESMKRKEDSYFNIRLRGFWPYAEMQNKIEFKLEQYGIKIRKVAPNNTSKTCSKCGHLNNYFNFEYRKKNKFPHFKCEKCNFKENADYNAALNISNPKLKSTKEEP

SEQ ID NO: 2080 - protein, 726 aa, synthetic construct
SEVEFSHEYWMRHALTLAKRARDEREVPVGAVLVLNNRVIGEGWNRAIGLHDPTAHAEIMALRQGGLVMQNYRLTDATLYVTFEPCVMCAGAMIHSRIGRVVFGVCNSKHGAAGSLMNVLNYPGMNHCVEITEGILVDECAALLCDFYRMPRQVLNAQKKAQSSISSGGSSGGSSGSVTPGASGSVTPKSSGSSSAGSTKDTITKTLKLRIVRPYNSAEVEKIVADEKNNREKIAMEKNKDKVKEACSKHLKVASYCTTQVERNACLFCKARKLDDKFYQKLRGQFPDAVFWQELGGIFRQLQKQAAEIYNQSLIELYYEIFIKGKGITNASRVEHYLSDVCYTRAAELFKNAAIASGLRSKVRSNFRLKELKNMKSGLPTTKSDNFPIPLVKQKGGQYTGFEISSHNDDFIIKIPFGRWQVRKEIDKYRPWEKFNFEQVRKSPKPISLLLSTQRRKRNKGWSKDEGTEAEIRKVMNGDYQTSYIEVKRGSKIGEKSAWMLNLSIDVPKIDKGVDPSIIGGIDVGVKSPLVCAINNALSRYSISDNDLFHFNKKMFARRRILLRKNRHKRAGHGARNKLKPITVLTEKSERFRKKLIERWACEIANFFIKNKVGTVQMENLESMKRREDSYFNIRLRGFWPYAEMQNKIEFKLKQYGIEIRKVAPNNTSKTCSKCGHPNNYFNFEFRKRNKFPHFKCEKCNFKENADYNAALNISNPKLKSTKEEP

SEQ ID NO: 2081 - protein, 726 aa, synthetic construct
SEVEFSHEYWMRHALTLAKRARDEREVPVGAVLVLNNRVIGEGWNRAIGLHDPTAHAEIMALRQGGLVMQNYRLTDATLYVTFEPCVMCAGAMIHSRIGRVVFGVRNSKRGAAGSLMNVLNYPDMNHCVEITEGILVDECAALLCDFYRMPRQALNAQKKAQSSISSGGSSGGSSGSETPGASESATPESSGGSSGGSAKNTITKTLKLRIVRPYNSAEVEKIVADEKNNREKIALEKNKDKVKEACSKHLKMAAYCTTQVERNACLFCKARRLDDKFYRKLRGQFSDAVFWQEIGEIFRQLQKQAAEIYNQSLIELYYEIFIKGKGFANASSVEHYLSDVCYTRAAELFKNAAIASGLRGKVKSNFRLKELKNMKSGLPTTKSDNFPIPLVKQKGGQYTGFEISSHNDDFIIKIPFGRWQVKKEIDKYRPWEKFDFEQVRKSPKPISLLLSTQRRKRNKGWSKDEGTEAEIRKVMNGDYQTSYIEVKRGSKIGEKSAWMLNLSIDVPKIDKGVDPSIIGGIDVGVKSPLVCAINNAFSRYSISDNDLFHYNKKMFARRRILLKRNRHKRAGHGAKNKLKPISILTEKSKRFRKKLIERWACEIADFFIKNKVGTVQIENLESMKRKEDSYFNIRLRGFWPYAEMQNKIEFKLKQYGIEIRKVAPNNTSKTCSKCGHLNNYFNFEYRKKNKFPHFKCKKCNFKENADYNAALNISNPKLKSTKEEP

SEQ ID NO: 2082 - protein, 726 aa, synthetic construct
SEVEFSHEYWMRHALTLAKRARDEREVPVGAVLVLNNRVIGEGWNRAIGLHDPTAHAEIMALRQGGLVTQNYRLIDATLYVTFEPCVMCAGAMVHSRIGRVVFGVRNSKRGAAGSLMNVLDYPGMGHRVEITEGILADECAALLCDFYCMPRQVFNAQKRAQSSINSGGSSGGSSGSETPGTSESATPESSGGGSSGSAKNTITKTLQLRIVRPYNSAEVERIVADEKNSREKIALEKNKDKVKEACSKHLKVAAYCTTQVERNACLFCKARKLDDKFYQKLRGQFPDAVFWQEIGEIFRQLQKQAAEIYNQSLIELYYEIFIKGKGFANASSVEHYLSDVCYTRAAELFKNAAIASGLRGKVKSNFRLKELKNMKSGLPTTKSDNFPIPLVKQKGGQYTGFEISSHNDDFIIKIPFGRWQEKKEIDKYRPWEKFDFEQVRKSPKPISLLLSTQRRKRNKGWSKDEGTEAEIRKVMNGDYQTSYIEVKRGSKTGEKSAWMLNLSIDVPKIDKGVDPSVIGGIDVGVKSPLVCAINNAFSRYSISDNDLFRFNKKMFARRRILLKKNRHKRAGHGARNKLKPITVLTEKSKRFRKKLIERWACEIANFFIKNKVGTVQMENLESMKRKEDSYFNIRLRGLWPYAEMQNKIEFKLKQYGIEIRKVAPNNTSKTCSKCGYLNNYFNFEYRKRNKFPHFKCEKCNFKENADYNAALNISNPKLKGTKEEP

SEQ ID NO: 2083 - protein, 726 aa, synthetic construct
SEVEFSHEYWMRHALTLAKRARDEREVPVGAVLVLNNRVIGEGWNRAIGLHDPTAHAEVMALRQGGLVMQNYRLIDATLYVTFEPCVMCAGAMVHSRIGRVVFGVRNSKRGAAGSLMNVLDHPGMGHRVEITEGILADECAALLCDFYCMPRQVFNAQKRAQPSIDSGGSFGGSSGSETPGTSESATPESSGGGSSGSAKNTITKTLQLRIVRPYNSAEVEKIVADEKNNREKIALEKNKDKVKEACSKHLKVASYCTTQVERSACLFCKARKLDDKFYQKLRGQFPDAVFWQEIGEIFRQLQKQAAEIYNQSLIELYYEILIKGKGFANASSVEHYLSDVCYTRAAELFKNAAIASGLRGKVKSNFRLKELKNMKSGLPTTKSDNFPIPLVKQKGGQYTGFEISSHHDDFIIKIPFGRWQVKKEIDKYRPWEKFDFEQVRKSPKPISLLLSTQRRRRDKGWSKDEGTEAEIRKVMNGDYQTSYIEVKRGSKTGEKSAWMLNLSIDVPKIDKGVDPSIIGGIDVGVKSPLVCAINDAFGRYSISDNDLFRFNKKMFARRRILLKKNRHKRAGHGAKNKLKPITIMTEKSKRFRKKLIERWACEIADFFIKNKVGTVQMENLESMKRKEDSYFNIRLRGFWPYAEMQNKIEFKLKQYGIVVRKVAPNNTSKTCSQCGHLNNYFNFEYRKKNQFPYFKCEKCNFKENADYNAALNISNPQLKSTKGEP

SEQ ID NO: 2084 - protein, 726 aa, synthetic construct
SEVELSHEYWMRRALTLAKRARDEREVPVGAVLVLNNRVIGVGWNRAVGLHDPTAHAEIMALRQGGLVMQNYRLIEATLYVTFEPCIMCAGAMIHSRIGRVVFGVRNSKRGAAGSLMNVLNYPGMNHRVEVTEGILADECAALLCDYYRMPRQVFNARKKAQSSINSGGPSGGSSGSETPGTSESATPESSGGGSSGSAKNTITKTLQLRIVRPYNSAEVEKIVADEKNNREKIALEKNKDKVKEACSKHLKVAAYCTTQVERDACLFCRARKLDDKFYQRLRGQFPDAVFWQEIGEIFRQLQKQAAEIYNQSLIELYYEIFIKGKGFANASSVEHYLSDVCYTRAAELFKNAAIASGLRGKVKSNFRLKELKNMKSGLPTTKSDNFPIPLVKQKGGQYTGFEISSHNDDFIIKIPFGRWQVKKEIDKYRPWEKFDFEQVRKSPKPISLLLSTQRRKRNKGWSKDEGTEAEVKKVMNGDYQISYIEVKRGSKIGEKSAWTLNLSIDVPKIDKGVDPSIIGGIDVGVKSPLVCAISDAFSRYSISDNDLFHFNKKMFARRRILLKKSKHKRAGHGVKNKLKPITILTEKSRRFRKKLIERWACEIADFFIKNKVGTVQMENLEGMKRKEDSYFNIRLRGFWPYAEMQNKIEFKLKQYGIEIRKVAPNNTSKTCSKCGHLNNYFNFEYRKKNKFPHFKCEKCNFKEDADYNAALNISNPKLKSTKEEP

SEQ ID NO: 2085 - protein, 726 aa, synthetic construct
SEVEFSHEYWMRHALTLAKRARDEREVPVGAVLVLNNRVIGEGWNRAIGLHDPTAHAEIMALRQGGLVMQNYRLIDATLYVTFEPCVMCAGAMIHSRIGRVVFGVRNNKHGAAGSLVNVLNYPGMNHRVEITEGILADECAALLCDFYRMPRQVLNAQKKAQSSISSGGSSGGSSGGKAPGTSESATLESSGGSSGGSAKNSITKTLKLRIVRPYNSAEVEKIVADEKNSREKIALERNKDKVKEACSEHLKVAAYCTTQVERNACLFCKARKLDDRFYQKLRGQFPDAVFWQEIGEIFRQLQKQAAEIYNQSLIELYYEIFIKGKGIANASSVEHYLSDVCYTRAAELFKNAAIASGLRNKVKSNFRLKELRSMKSGLPTTKSDNFPIPLVKQKGGQYTGFEISNHNSDFIIKIPFGRWQVKKEIDKFRPWEKFDFEQVRKSPKPISLLLSTQRRKRNKGWGRDEGTEAEIKKVMNGDYQTSYIEVKRSSKIGEKGAWMLSLSIDVPKIDKGVDPSIVGGVDVGVKSPLVCAINNALSRYSISDNDLYRFNKKMFARRRILLKKNRHKRAGHGAKNKLKPITILTEKSERFRKKLIERWACEIADFFIKNKVGTVQMENLEGMKRKEDSYFNIRLRGLWPYAEMQNKIEFKLKQYGIEIRKVAPNNTSKTCSKCGHLNNYFNFEYRKKNKFPHFKCEKCNFKENADYNAALNISNPKLRSTKEEP

SEQ ID NO: 2086 - protein, 726 aa, synthetic construct
SGDEFSHEYWMRHALTLAKRARDGREVPVGAVLVLNNRVIGEGWNRAIGLHDPTAHAEIMALRQGGLVMQNYRLIDATLYVTFEPCVMCAGAMVHSRIGRVVFGVRNSKRGAAGSLMNVLDYPGMGHRVGITGGILADECAALLCDFYRMPHQVFNAQKKAQSSINSGGSSGGSSGSVTPGPSESATPESSGGSSGSSAKNTITKTLQLRIVRPYNSAEVEKIVADEKNNREKIALEKNKDKVKEACSKHLKVASYCTTQVERNACLFCKARKLDDKFYQRLRGQFPDAVFWQELGEIFRQLQKQAAEIYNQSLIELYYEIFIKGKGFANASSVEHYLSDVCYTRAAELFKNAAIASGLRGKVKSNFRLKELKNMKSGLPTTKSDNFPIPLVKQKGGQYTGFEVSSHNDDFVIKIPFGRWQVKKEIDKYRPWEKFDFEQVRKSPKPISLLLSTQRRKRNKGWSRDEGTEAEVRKVMNGDYQTSYIEVKRGSKIGEKSAWMLNLSIDVPKIDKGVDPSIIGGIDVGVKSPLVCAVNNALSRYSISDNDLFHFNKKMFARRRILLRKNRHKRAGHGAKNKLKPITIMTEKSKRFRKKLIERWACEIADFFIKNKVGTVQMENLESMKRKEDSYFNIRLRGFWPYAEMQNKIEFKLKQYGIVVRKVAPNNTSKTCSKCGHLNNYFNFEYRKKNKFPHFKCEKCNFKEDADYNAALNISNPKLKSTKGEP

SEQ ID NO: 2087 - protein, 726 aa, synthetic construct
SEVEFSHEYWMRHALTLAKRARDEREVPVGAVLVLNDRAIGEGWNRAIGLHDPTAHAEIMALRQGGLVTQNYRLIDATLYVTFEPCVMCAGAMIHSRIGRVVFGVRNSKHGAAGSLVNVLNYPGMNHRVEITEGVLADECAALLCDFYRMPRQVFNARKKAQSNINPGGSSGGSSGSETPGTSDSATPGSSGGSSGGSAKNTITKTLKLRIVRPYNSAEVEKIVADEKNNREKTALEKNKDKVKEACSEHLKVATYCTTQVERNACLFCKARKLDDKFYQKLRGQFPDAVFWQEIGEIFRQLQKQAAEIYNQSLIELYYEIFIKGKGFANASSVEHYLSDVCYTRAAELFKNAAIASGLRNKTKSNFRLKELRSMKSGLPTTKSDNFPIPLVRQKGGQYTGFEISSHNDDFIIKIPFGRWQVKEEIDKYRPWEKFDFEQVRRNPKPISLLLSTQRRKRNKGWSKDEGTEAEIRKVMNGDYQTSYIEVKRGSKIGEKSAWMLNLSIDVPKIDKGVDPSTIGGIDVGVKSPLVCAINNAFCRYSISDNDLFHFNKKMFARRRILLKKSRHKRAGHGAKNKLKPISILTEKSKRFRKKLIERWACEIADFFIKNKVGTVQMENLESMKRKEDSYFNIRLRGFWPYAEMQNKIEFKLKQYGIVVRKVAPNNTSKTCSQCGHLNNYFNFEYRKKNKFPYFKCEKCNFKENADYNAALNISNPQLKSTKGEP

SEQ ID NO: 2088 - protein, 726 aa, synthetic construct
SEVEFSHEYWMRRALTLAKRARDEREVPVGAVLVLNNRVIGVGWNRAAGLHDPTAHAEIMALRQGGLVMQNYRLVEATLYVTFEPCVMCAGAMVHSRIGRVVFGVRNNKRGAAGSLMNVLNYPGMNHRVEITEGILADECAALLCDFYRMPRQVLNAQKKARSCINSGGSSGGSSGSETPGTSESATPESSGGSSGGSAKNTITKTLKLRIVRPYNSAEVEKIVADEKDNRERIALEKNKGKVKEACSKHLKVAAYCTTQVERNACLFCKARRLDDKFYQKLRGQFPDAVFWQEIGEIFRQLQKQAAETYNQSLIELYYEIFIKGKGIANASSVEHYLSDVCYTRAAELFKNAAIASGLRNKVKSNFRLKELRSMKSGLPTTKSDNFPIPLVRQKGGQYTGFEISNHNSDFIIKIPFGRWQAKKEIDKYRPWEKFDFEQVRKSPKPISLLLSTQRRKRNRGWSKDESTEAEIKKVMNGDYQTSYIEVKRGSKTGEKSAWMLNLSIDVPKIDKGVDPSIIGGIDVGVKSPLVCAINNAFSRYSISDNDLFRFNKKMFARRRILLRKNRHKRAGHGAKNKLKPISILTGKSERFRKKLIERWACEIADFFIKNKVGTVQMENLESMKRKEDSYFNIRLRGFWPYAEMQNKIEFKLKQYGIKIRKVAPNNTSKTCSKCGHLNNYFNFEYRKKNKFPHFKCEKCNFKENADYNAALNISNPKLKSTKEEP

SEQ ID NO: 2089 - protein, 726 aa, synthetic construct
SEDEFSHEYWMRHALTLAKRARDGREVPVGAVLVLNNRVIGEGWNRAIGLHDPTAHAEIMALRQGGLVMQNYRLIDATLYVTFEPCVMCAGAMVHSRIGRVVFGVRNSKRGAAGSLMNVLDYPGMGHRVEITEGILADECAALLCDFYCMPRQVFNAQKRAQSSINSGGSSGGSSGSETPGTSESATPESSGGGSSGSAKNTITKTLQLRIVRPYNSAEVEKIVADEKNNREKIALEENKDKVKEACSKHLKVASYCTTQVERNACPFCKARKLDDKFYQKLRGQFPDAVFWQELGEILRQLQKQAAEIYNQSLIELYYEIFIKGRGFANASSVEHYLSGVCYTRAAELFRNAAIASGLRGKVKSNFRLKELKNMKSGLPTTKSDNFPIPLVKQKGGQYTGFEISSHNDDFIIKIPFGRWQVKKEIDKYRPWEKFDFEQVRKSPKPISLLLSTRRRKRNKGWSKDEGTEAEIRKVMNGDYRTSYIEVKRGSKTGEKSAWMLNLSIDVPKIDKGVDPSIIGGIDVGVKSPLVCAINNAFSRYSISDNDLFRFNKKMFARRRILLKKNRHKRAGHGAKNKLKPISILTEKSERFRKKLIERWACEVADFFIKNKVGTVQMENLESIKRKEDSYFNIRLRGFWPYAEMQNRIEFKLKQFGIEIRKVAPNNTSKTCSKCGHLNNYFNFEYRKKNKFPHFKCEKCNFKENADYNAALNISNPKLKSTKEEP

SEQ ID NO: 2090 - protein, 726 aa, synthetic construct
SGVEFSHEYWMRHALTLAKRARDEREVPVGAILVLNNRVIGEGWNRAIGLHDPTAHAEIMALRQGGLVTQNYRLIDATLYVTFEPCVMCAGAMIHSRIGRVVFGVRNSKHGAAGSLVNVLNYPGMNHRVEITEGILADECAALLCDFYRMPRQVFNARKKAQSSINPGGSSGGSSGSETPGTSESATPESSGGSSGSSAKNTITKTLQLRIVRPYNSAEVEKIVADEKNNREKIALEKNKDKVKEACSKHLKVAAYCTTQVERNACLFCKARKLDDKFYQKLRGQFPDAVFWQEVSEIFRQLQKQAAEIYNQSLIELYYEIFIKGKGFANASSVEHYLSDVCYTRAAELFKNAAIASGLRGKVKSNFRLKELKNMKSGLPTTKSDNFPIPLVKQKGGQYTGFEISSHNDDFIIKIPFGRWQVKKEIDKYRPWEKFDFEQVRKSPKPVSLLLSTQRRKKNKGWSKDEGTEAEIRRVMNGDYQTSYIEVKRGSKIGERSAWMLNLSIDVPKIDKGVDPMIIGGVDVGVKSPLVCAINNAFSRYSISDNDLFRFNKKMFARRRILLKKNRHKRAGHGAKNKLKPISILTEKSKRFRKKLIERWACEIADFFIKNKVGTVQMENLESMKRKEDSYFNIRLRGLWPYAEMQNKIEFKLKQYGIKIRKVAPNNTSKTCSKCGHLNNYFNFEYRKKNKFPHFKCERCSFKENADYNAALNISNPKLRSTKEEP

SEQ ID NO: 2091 - protein, 726 aa, synthetic construct
SEVEFSHEYWMRHALTLAKRARDEREVPVGAVLVLNNRVIGEGWNRAIGLHDPTAHAEIMALRQGGLVMQNYRLTDATLYVTFEPCVMCAGAMIHSRIGRVVFGVRNSKRGAAGSLMNVLNYPGMNHCVEITEGILVDECAALLCDFYRMPRQVLNAQKKAQSSISSGGSSGGSSCSETPGASESVTPKSSGGSSAGSTKNTITKTLKLRIVRPYNSAEVEKIVADEKNSREKIALEKNKDKVKEACSEHLKVAAYCTTQVERNACLFCKARKLDDRFYQKLKGQFPDAVFWQEIGEIFRQLQKQAAEIYNQSLIELYYEIFIKGKGFANASSVEHYLSDVCYTRAAELFKNAAIASGLRGKVKSNFRLKELKNMKSGLPTTKSDNFPIPLVKQKGGQYTGFEVSSHNDDFIIKIPFGRWQVKKEIDKYRPWEKFDFEQVRKSPRPISLLLSTQRRKRNKGWSKDEGTEAEIRKVMNGDYQTSYIEVKRGSKIGERSAWMLNLSIDVPKIDKGVDPSIIGGIDVGVKSPLVCAINNAFSRYSISDNDLFRFNKKMFARRRILLKKSKHKRAGHGAKNKLKPITILTEKSGRFRKKLIERWACEIADFFIKNKVGTVQMENLESMKRREDSYFNIRLRGFWPYAEMQNKIEFKLKQYGIEIRKVAPNNTSKTCSKCGHLNNYFNFEYRKKNKFPHFKCEKCNFKENADYNAALNISNPKLKSTKEES

SEQ ID NO: 2092 - protein, 726 aa, synthetic construct
SEVEFSHEYWMRHALSLAKRARDEREVPVGAVLVLNNRIIGEGWNRAIGLHDPTAHAEIMALRQGGLVTQNYRLTDATLYVTFEPCVMCAGAMIHSRIGRVVFGVRNSKHGAAGSLMNVLNYPGMNHRVEITEGTLADECAALLCDFYRMPRQVFSARKKAQSSINSGGSSGGNSGSKTPGTSESATPESSGGSSGGSAKNTITKTLKLRIVRPYNSAEVEKIVADEKNNREKIALEKNKDKVKEACSKHLKVAAYCTTQVERNACQFCKARKLDDKFYQKLRGQFPDAVFWQEIGEIFRQLQKQAAEIYNQSLVELYYEIFIKGKGFANASSAEHYLSDVCYTRAAELFKNAAIASGLRGKVKSNFRLKELKNMKSGLPTTKSDNFPIPLVKQKGGKYTGFEISSHNNDFIIKIPFGRWQVKKEIDKYRPWEKFDFEQVRKSPKPISLLLSTQRRKRNKGWSKDEGTEAEIRKVMNGDYQTSYIEVKRGSKIGEKSAWMLNLSIDVPKIDKGVDPSIIGGIDVGVKSPLVCAINNAFSRYSISDNELFHFNKKMFARRRILLKKNRHKRAGHGAKNKLKPISVLTEKSGRFRKKLIERWACEIADFFIKNKVGTVQMENLGSMKRKEDSYFNIRLRGFWPYAEMQNKIEFKLKQYGIEIRKVAPDNTSKTCSKCGHLNNYFNFEYRKKNKFPHFKCERCNFKEDADYNAALNISNPKLKSTKEEP

SEQ ID NO: 2093 - protein, 726 aa, synthetic construct
SEVEFSHEYWMRHALTLAKRARDEREVPVGAILVLNNRAIGEGWNRAIGLHDPTAHAEIMALRQGGLVMQNYRLIDATLYVTFEPCAMCAGAMIHSRIGRVVFGVRNSKHGAAGSLMNVLNYPGMNHRVEITEGILADECAALLCDFYRMPRLVFNARKKTQSSINPGGSSGGSSGSETPGTSESAAPESSGGSSGSSAKNTITKTLKLRIVRPYNSAEVEKIVADEKNNREKIALEKNKDKVKEACSKHLKVAAYCTTQVERNACLFCKARRLDDKFYQKLRGQFPDAVFWQEIGEIFRQLQKQAAEIYNQSLIELYYEIFIKGKGIANASSVEHYLSDVCYTRAAELFKNAAIASGLRNKVKSNFRLKELRSMRSGLPTTKSDNFPIPLVRQKGGQYTGFEISNHNSDFIIKIPFGRWQAKKEIDKYRPWEKFDFEQVRKSPKPISLLLSTQRRKRNRGWSKDESTEAEIKKVMNGDYQTSYIEVKRGSKTGEKSAWMLNLSIDVPKIDKGVDPSIIGGIDVGVKSPLVCAINNAFSRYSISDNDLFRFNKKMFARRRILLKKNRHKRAGHGAKNKLKPISILTGKSERFRKKLIERWACEIADFFVKNKVGTVQMENLESMKGKEDSYFNIRLRGFWPYAEMQNKIEFKLKQYGIKIRKVAPNNTSKTCSKCGHLNDYFNFEYRRKNKFPHFKCEKCYFKEDADYNAALNISNPKLKSTKEEP

SEQ ID NO: 2094 - protein, 726 aa, synthetic construct
SEVEFSHEYWMRHALTLAKRARDEREVPVGAVLVLNNRVIGEGWNRAIGLHDPTAHAEIMALRQGGLVMQNYRLSDATLYVTFEPCVMCAGAMVHSRIGRVVFGVRNSKRGAAGSLMNVLNHPGMSHRVEITGGILADECAALLCDFYRMPRQVFNAQKKARSNINSGGSSGGSSGSETPGTSESATPESSGGSSGGSAKNTITKTLQLRIVRPYNSAEVEKIVTDEKNNREKIALEKNKDKVKEACSKHLKMASYCTTQVERNACLFCKARKLDDKFYQKLRGQFPDAVFWQELGGIFRQLQKQAAEIYNQSLIELYYEIFIKGKGITNASRVEHYLSDVCYTRAAELFKNAAIASGLRSKVRSNFRLKELKNMKSGLPTTKSDNFPIPLVKQKGGQYTGFEISSHNSDFIIKIPFGRWQEKEEIGKYRPWEKFDFEQVRRSPKPISLLLSTQRRKRNKGWSKDEGTEAEIRKVMNGDYQTSYIEVKRGSKTGEKSAWMLNLSIDVPKIDKGVDPSIIGGIDVGVKSPLVCAINNALSRYSISDNDLYRFNKKMFARRRILLKKSKHKRAGHGAKNKLKPITILTEKSGRFRKKLIERWACEIADFFIKNKVGTVQMENLEGMKRKEDSYFNIRLRGFWPYAEMQNKIEFKLKQYGIEIRKVAPNNTSKTCSKCGHLNNYFNFEYRKKNKFPHFKCEKCNFKENADYNAALNISNPMLKSTKEEP

SEQ ID NO: 2095 - protein, 726 aa, synthetic construct
SEVEFSHEYWMRHALTLAKRARDEREVPVGAVLVLNNRVIGEGWNRAIGLHDPTAHAEIMALRQGGLVMQNYRLTDATLYVTFEPCVMCAGAMIHSRIGRVVFGVRNSKYGAAGSLVNVLNYPGMNHRVEITEGILADECAALLCDFYRMSRQVFNARKKAQPSINPGGSSGGGSGSETPGTSESATPESSGGSSAGSTKNTITKTLKLRIVRPYNSAEVEKIVADEKNSREKIALEKNRDKVKEACSEHLKVAAYCTTQVERSACLFCKARKLDDKFYQKLRGQFPDAVFWQEIGEIFRQLQKQAAEIYNQSLIELYYEIFIKGKGFANASSVEHYLSDVCYTRAAELFKNAAIASGLRGKVKSNFRLKELKNMKSGLPTTKSDNFPIPLVKQKGGQYTGFEISSHNDDFIIKIPFGRWQVKKKIDKYRPWEKFDFEQVRKSPKPISLLLSTQRRKRNKGWSKDEGTEAEIRKVMNGDYQTSYIEVKRGSKIGEKSAWMLNLSIDVPKIDKGVDPSIIGGIDVGVKSPLVCAINNAFSRYSISDNDLFHFNKKMFARRRILLKKNRHKRAGHGAKNKLKPITILTEKSVRFRKKLIERWACEIADFFIKNKVGTVQMENLESMKGKEDSYFNIRLRGFWPYAEMQNKIEFKLKQYGIEIRKVAPNNTSKTCSKCGHLNNYFNFEYRKKNKFPHFKCEKCYFKEDADYNAALNISNPRLKSTKEEP

SEQ ID NO: 2096 - protein, 726 aa, synthetic construct
SGVEFSHEYWMRHALTLAKRARDEREVPVGAILVLNNRVIGEGWNRAIGLHDPTAHAEIMALRQGGLVMQNYRLIDATLYVTFEPCVMCAGAMIHSRIGRVVFGVRNSKHGAAGSLVNVLNYPGMNHRVGITEGILADECAALLCDFYRMPRQVFNARKKAQSSINPGGSSGGSSGSETQGTSESATPESSGGSSGGSAKNTITKALKLRIVRPYNSAEVEKIVADEKNNRERIALEKNKDKVKEACSKHLKVAAYCTTQVERNACLFCKARKLDDKFYQKLRGQFPDAVFWQEIGEIFRQLQKQAAEIYNQSLIELYYEIFIKGKGFANASSVEHYLSDVCYTRAAELFKNAAIASGLRGKVKSNFRLKELKNMKSGLPTTKSDNFPIPLVKQKGGQYTGFEISSHNDDFVIKIPFGRWQVKKEIDKYRPWEKFDFEQVRKGPKPISLLLSTQRRKRNKGWSKDEGTEAEIRKVMNGDYRTSYIEVKRGSKTGEKGAWMLNLSIDVPKIDKGVDPSIIGGIDVGVKSPLVCAINNAFSRYSISDNDLFRFNKKMFARRRILLKKNRHKRAGHGAKNKLKPISILTGKGERFRKKLIERWACEIADFFIKNKVGTVQMENLESMKRKEDSYFNIRLRGFWPYAEMQNKIEFKLKQYGIEIRKVAPNNTSKTCSKCGHVNNYFNFEYRKKNKFPHFKCEKCNFKENADYNAALNISNPRLKSTKEEP

SEQ ID NO: 2097 - protein, 726 aa, synthetic construct
SEVEFSHEYWMRHALTLAKRARDEREVPVGAVLVLNNRVIGEGWNRAIGLHDPTAHAEIMALRQGGLVMRNYRLTDATLYVTFEPCIMCAGAMIHSRIGRVVFGVRNSKRGAAGSLMNVLNYPGMNHCVEITEGILVDECAALLCDFYRMPRQVLNARKKAQSSISPGGSSGGSSGSETPGASESVTPKSSGGSSGSSAKNTITKTLKLRIVRPYNSAEVEKIVADEKNNREKIALEKNKGKVKEACSKHLEVAAYCTTQVERNTCLFCKARKLDDKFYQKLRGQFPDAVFWQELGEIFRQLQKQAAEIYNQSLIELYYEIFIKGKGFANASSVEHYLSDVCYTRAAELFKNAAIASGLRGKVKSNFRLKELKNMRSGLPTTKSDNFPIPLVKQKGGQYTGFEISSHNDDFIIKIPFGRWQVKEEIDKYRPWEKFDFEQVRKNPKPINLLLSTLRRKRNKGWSKDEGTEAEIRKVMNGDYQTSYIEVKRGSKTGEKSAWMLNLSIDVPKIDKGVDPSIIGGIDVGVKSPLVCAINNAFSRYSISDNDLFRFNKKMFARRRILLKKNRHKRAGHGAKNKLKPISILTEKSKRFRKKLIERWACEIADFFIKNKVGTVQMENLESMKRKEDSYFNIRLRGFWPYAEMQNKIEFKLKQYGIEIRKVAPNNTSKTCSKCGHLNNYFNFEYRKKNKFPHFKCEKCNFKENADYNAALNISNPKLKSTKEEP

SEQ ID NO: 2098 - protein, 726 aa, synthetic construct
SEVEFSHEYWMRHALTLAKRARDEREVPVGAVLVLNNRVIGEGWNRAIGLHDPTAHAEIMALRQGGLAMRNYRLVDATLYVTFEPCVLCAGAMVHSRIGRVVFGVRNSKRGAAGSLMNVLNHPGMNHRVEITGGILADECAALLCDFYRMPRQVFNAQKKARSNINSGGSSGGSSGSETLGTSESATPESSGGSSGGSAKNTITKTLKLRIVRPYNSAEVEKIVADEKNNREKIALEKNKDKVKEACSEHLKVAAYCTTQVERNACLFCKARKLDDKFYQKLRGQFPDAVFWQEIGEIFRQLQKQAAEIYNQSLIELYYEIFIKGKGFANASSVEHYLSDVCYTRAAELFKNAAIASGLRSKIKSNFRLKELKNMKSGLPTTKSDNFPIPLVKQKGGQYTGFEISDHNSDFIIKIPFGRWRVKKEIDKYRPWEKFDFEQVRKSPKPISLLLSTQRRKRNKGWSRDEGTEAEIKKVMNGDYQVSYIEVKRGSKIGEKSAWMLNLSIDVPKIDKGVDPSIIGGIDVGVKSPLVCAINNAFSRYSISDNDLFHFNKKVFARRRILLKKNRYKRASHGAKNKLKPITILSEKSERFRKKLIEKWACEIADFFIRNKVGTVQMENLESMKRKEDGYFNIRLRGFWPYAEMQNKIELKLKQYGIEIRKVAPNNTSKTCSKCGHLNNYFNFEYRKKNKFPHFKCEKCNFKENADYNAALNISNPKLKSAKEEP

SEQ ID NO: 2099 - protein, 726 aa, synthetic construct
SEVEFSHEYWMHHALTLAKRARDEREVPVGAVLVLNNRVIGVGWNRAIGLHDPTAHAEIMALRQGGLVTQNYRLVDATLYVTFEPCVMCAGAMIHSRIGRVVFGVRNNKHGAAGSLVNVLDYPGMNHRVEITEGILADECAALLCDFYRMPRQVFSARKKAQSSISSGGPSGGSSCSETPGASESVTPKSSGGSSTGSTKNTITKTLKLRIVRPYNSAEVEKIVADEKNSREKIALEKNKDKVKEACSEHLKVAAYCTTQVERNACLFCKARRLDDKFYQKLRGQFPDAVFWQEIGEIFRQLQKQAAETYNQSLIELYYEIFIKGKGIANASNVEHYLSDVCYTRAAELFKNAAIASGLRNKIKSNFRLKELRNMKSGLPTTKSDNFPIPLVKQKGGQYTGFEISNHNSDFIIKIPFGRWQAKKEIDKYRPWEKFDFEQVRKSPKPISLLLSTQRRKRNRGWSKDEGTEAEVKKVMNGDYQISYIEVKRGSKIGEKSAWTLNLSIDVPKIDKGVDPSIIGGIDVGVKSPLVCAISNAFSRYSISDNDLFHFNKKMFARRRILLKKSKHKRAGHGVKNKLKPITILTEKSRRFRKKLIERWACEIADFFIKNKVGTVQMENLEGMKRKEDSYFNIRLRGFWPYAEMQNKIEFKLKQYGIEIRKVAPNNTSKTCSKCGHLNNYFNFEYRKKNKFPHFKCEKCSFKENADYNAALNISNPKLKSTKEEP

SEQ ID NO: 2100 - protein, 726 aa, synthetic construct
SEVEFSHEYWMRHALTLAKRARDEREVPVGAVLVLNNRVIGVGWNRAIGLHDPTAHAEIMALRQGGLVMQNYRLTDATLYVTFEPCVMCAGAMIHSRIGRVVFGVRNSKRGAAGSLVNVLSYPGMNHCVEITEGILVDECAALLCDFYRMPRQVLNAQKKVQSSISSGGLSGGSSGSETPGVSESVTPKSSVGSSASSTKNTITKTLKLRIVRPYNSAEVEKIVADEKNNREKIALEKNKDKVKEACSKHLKVAAYCTTQVERNACLFCKARRLDDKFYQKLRGQFPEAVFWQEIGEIFRQLQKQAAEIYNQSLIELYYEIFIKGKGFANASSVEHYLSDVCYTRAAELFKNAAIASGLRGKVKSNFRLKELKNMKSGLPTTKSDNFPIPLVKQKGGQYTGFEISNHNSDFIIKIPFGRWQAKKEIVKYRPWEKFDFEQVRKSPKPISLLLSTQRRKRNKGWSKDEGTEAEIRKVMNGDYQTSYIEVKRGSKTGEKSAWMLNLSIDVPKIDKGVDPSIIGGIDVGVKSPLVCAINNALSRYSISDNDLFRFNKKMFARRRILLKKNRHKRAGHGAKNKLKPISILTGKSERFRKKLIERWACEIADFFIKNKVGTVQIENLESMKRKEDSYFNIRLRGFWPYAEMQNKIEFKLKQYGIEIRKVAPNNTSKTCSKCGHLNSYFNFEYRKKNKFPHFKCEKCNFKENADYNAALNISNPKLKSTKEEP

SEQ ID NO: 2101 - protein, 726 aa, synthetic construct
SEIEFSHEYWMRHALTLAKRARDEREVPVGAVLVLNNRVIGEGWNRAIGLHDPTAHAEIMALRRGGLVMQNYRLTDATLYVTFEPCVMCAGAMIHSRIGRVVFGVRNSKRGAAGSLMNVLNYPGMNHCVEITEGILADECAALLCDFYCMPRQVFNAQKRAQSSINSGGSSGGSSGSETPGTSESATPESSGGGSSGSAKNTITKTLQLRIVRPYNSAEVEKIVADEKNNREKIALEKNKDKVKEACSKHLKVASYCTTQVERNACPFCKARKLDDKFYQKLRGQFPDAVFWQELGEIFRQLQKQAAEIYNQSLIELYYEIFIKGKGLANASSVEHYLSDVCYTRAAELFKNAAIASGLRGKVKSNFKLKELKSMKSGLPSTKSDNFPIPLVKQRGGQYTGFEISSHNDDFIIKIPFGRWQAKKEIDKYRPWEKFDFEQVRKSPKPISLLLSTQRRKRNRGWSKDEGTEAEIRKVMNGDYQTSYIEVKRGSKIGEKSAWMLNLSIDVPKIDKGVDPSIIGGIDVGVKSPLVCAINNAFSRYSISDNDLFHFNKKMFARRRILLRKNRHKRTGHGAKNKLKPITIMTEKSKRFRKKLIERWACEIADFFIKNKVGTVQMENLESMRRKEDSYFNIRLRGFWPYAEMQNKIEFKLKQYGIVVRKVAPNNTSKTCSKCGHLNNYFNFEYRKKNKFPHFKCEKCNFKENADYNAALNISNPKLKSTKEEP

SEQ ID NO: 2102 - protein, 726 aa, synthetic construct
SEVEFSHEYWMRHALALAKRARDEREVPVGAILVLNNRVIGEGWNRAIGLHDPTAHAEIMALRQGGLVMQNYRLIDATLYVTFEPCVMCAGAMIHSRIGRVVFGVRNSKHGAAGSLVNVLNYPGMNHRVEITEGILADECAALLCDFYRMPRQVFNARKKAQSSINPGGSSGGSSGSETPGTSESATPESSGGSSGGSAKNTITKTLKLRIVRPYNSTEVEKIVADEKNNREKIALEKNKGKVKEACSKHLKVAAYCTTQVERNACLFCKARRLDDKFYQKLRGQFPDAVFWQEIGEIFRQLQKQAAEIYNQSLIELYYEIFIKGKGIANASSVGHYLSDVCYTRAAELFKNAAIASGLRGKVKSNFRLKELKNMKSGLPTTKSDNFPIPLVKQKGGQYTGFEISSHNDDFIIKIPFGRWQVKKEIDKYRPWEKFDLEQVRKSPKPISLLLSTQRRKRNKGWSKDEGTEAEIRKVMNGDYQTSYIEVKRGSRIGEKSAWMLSLSIDVPKIDRGVDPSIIGGIDVGVKSPLVCAINNALSRYSISDNDLFHFNKKMFARRRILLKKNRHRRAGHGARNKLKPITVLTEKSKRFRKKLIERWACEIASFFVKNKVGTVQMENLESMKRKEDSYFNIRLRGLWPYAEMQNKIEFKLKQYGIKIRKVAPNSTSRTCSKCGHLNNYFNFEYRKKNKFPHFKCEKCNFKENADYNAALNISNPKLKSPKEES

SEQ ID NO: 2103 - protein, 726 aa, synthetic construct
SEVEFSHEYWMRHALTLAKRARDEREVPVGAVLVLNNRVIGEGWNRAIGLHDPTAHAEIMALRQGGLVMQNYRLVDATLYVTFEPCVMCAGAMIHSRIGRVVFGVRNSKRGAAGSLMNVLNYPGMNHCVEITEGILVDECAALLCDFYRMPRQVLNAQKKAQSSISSGGSSGGSSGSETPGASGSVIPKSSGGSSAGSTKDTITKTLKLRIVRPYNSAEVEKVVADEKNNREKIAMEKNKDKVKEACSKHLKVASYCTTQVERNACLFCKARKLDDKFYQKLRGQFPDAVFWQELGGIFRQLQKQAAEIYNQSLIELYYEIFIKGKGITNASRVEHYLSDVCYTRAAELFKNAAIASGLRSKVRSNFRLKELKNMKSGLPTTKSDNFPVPLVKQKGGQYTGFEISNHNSDFIIKIPFGRWQAKEEIDKYRPWERFDFEQVRKSPKPISLLLSTQRRKRNRGWSKDEGTEAEIRKVMNGDYQTSYIEVKRGGKIGEKSAWMLNLSIDVPKIDKGVDPSIIGGIDVGVKSPLVCAINNAFSRYSISDNDLFRFNKKVFARRRILLKKNRHKRAGHGAKNKLKPITILTEKSKRFRKKLIERWACEIADFFIRNKVGTVQMENLESMKRKEDSYFNIRLRGFWPYAEMQNKIEFKLKQYGIKIRKVAPNNTSRTCSKCGHLNNYFSFEYRKKNKFPHFKCEKCNFKEDADYNAALNISNPKLKGTKEEP

SEQ ID NO: 2104 - protein, 726 aa, synthetic construct
SEVEFSHEYWMRHALTLAKRARDEREVPVGAVLVLNNRVIGEGWNRAIGLHDPTAHAEIMALRQGSLVMQNYRLTDATLYVTFEPCVMCAGAMIHSRIGRVVFGVRNSKRGAAGSLMNVLNCPGMNHCVEITEGILVDECAALLCDFYRMPRQVFNARKKAQSSINPGGSSGGSSGSETPGTSESATPESSGGSSGSSAKNTITKTLKLRIVRPYNSAEVEKIVADEKNNREKIALEKNKDKVKEACSKHLKVAAYCTTQVERNACLFCKARKLDDKFYQKLRGQFPDAVFWQEIGEIFRQLQKQAAEIYNQSLIELYYEIFIKGRGFANAGSVEHYLSDVCYTRAAELFKNAAIASGLRGKVKSNFRLKELKNMKSGLPTTKSDNFPIPLVKQKGGQYTGFEISSHNDDFIIKIPFGRWQVRKEIDKYRPWEKFDFEQVRKSPKPISLLLSTQRRKRNKGWSKDEGTEAEIRKVMNGDYQTSYIEVKRGSKIGEKSAWMLNLSIDVPKIDKGVDPSIIGGIDVGVKSPLVCAINNAFSRYSISDNDLFHFNKKMFARRRILLKKNRHKRAGHGAKNKLRPITILAEKSERFRKKLIEKWACEIADFFIKNKVGTVQMENLESMKRKEDSYFNIRLRGFWPYAEMQNKIEFKLKQYGIEIRKVAPNNTSKTCSKCGHLNNYFNFEYRKKNKFPHFKCEKCNFKENADYNAALNISNPKLKSTKEEP

SEQ ID NO: 2105 - protein, 726 aa, synthetic construct
SEVEFSHEYWMRHALALAKRARDEREVPVGAVLVLNNRAIGEGWNRAIGLHDPTAHAEIMALRQGGLVMQNYRLTDATLYVTFEPCVMCAGAMIHSRIGRVVFGVRNSKRGAAGSLMNVLNYPGMNHCVEITEGILVDECAALLCDFYRMPRQVLNAQKKAHSSINSGGSSGGSSGSVTPGTSESATPESSGGGFGGSAKNTITKTLQLRIVRPYNSAEVEKIVADEKNNREKTALEKNKDKVKEACSKHLKVAAYCTTQVERNACLFCKARKLDDKFYQKLRGQFPDAVFWQEVGEIFRQLQKQAAEIYNQSLIELYYEIFIKGKGFANASSVEHYLSDVCYTRAAELFKNAAIASGLRGKVKSNFRLKELKNMKSGLPTTKSDNFPIPLVKQKGGQYTGFEISNRNSDFIIKIPFGRWQVKKEINKYRPWEKFDFEQVRKSPKPISLLLSTQRRKRNKGWSRDEGTEAEIRKVMNGDYQTSYIEVKRGSKTGEKSAWMLNLSIDVPKIDKGVDPCIIGGIDVGVKSPLVCAINNALSRYSISDNDLFHFNKKMFARRRILLRKNRHKRAGHGAKNKLKPITIMTEKSKRFRKKLIERWACEIADFFTKNKVGTVQMENLESMKRREDSYFNIRLRGFWPYAEMQNKIEFKLKQYGIVVRKVAPNNTSKTCSKCGHLNNYFNFEYRKKNKFPHFKCEKCNFKEDADYNAALNISNPKLKSTKGEP

SEQ ID NO: 2106 - protein, 726 aa, synthetic construct; identical to SEQ ID NO: 684

SEQ ID NO: 2107 - protein, 726 aa, synthetic construct
SEVEFSHEYWMRHALTLAKRARDEREVPVGAVLVLNNRVIGEGWNRAIGLHDPTAHAEIMALRQGGLVMQNYRLIDATLYVTFEPCVMCAGAMIHSRIGRVVFGVRNNKHGAAGSLVNVLNYPGMNHRVEITEGILADECAALLCDFYRMPRQVFNARKKAQSSINSGGSSGGSSGSETPGTSESATPESSGGGSSGSAKNTITKTLQLRIVRPYNSAEVEKIVADEKNNREKIALEKNKDKVKEACSKHLKVASYCTTQVERSACPFCKARKLDDKFYQKLGGQFPDAVFWQELGEILRQLQKQAAEIYNQSLIELYYEIFIKGRGFANASSVEHYLSDVCYTRAAELFKNAAIASGLRGKVKSNFRLKELKNMKSGLPTTKSDNFPIPLVKQKGGQYTGFEISNHDGDFIIKIPFGRWQVKKEINKHRPWEKFDFEQVRRSPKPISLLLSTQRRKRNKGWSKDEGTEAEIRKVMNGDYQTSYIEVKRGSKIGEKSAWMLNLSIDVPKIDKGVDPSIIGGIDVGVKSPLVCAINNALSRYSISDNDLFHFNKKMFARRRILLRKNRHKRAGHGAKNKLKPITIMTEKSKRFRKKLIERWACEIADFFIKNKVGTVQMENLESMKRREDSYFNIRLRGFWPYAEMQNKIEFKLKQYGIVVRKVAPNNTSKTCSKCGHLNNYFNFEYRKKNKFPHFKCEKCNFKEDADYNAALNISNPKLKSTKGEP

SEQ ID NO: 2108 - protein, 726 aa, synthetic construct
SEVEFSHEYWMRHALTLAKRARDEREVPVGAVLVLNNRVIGEGWNRAIGLHDPTAHAEIMALRQGGLVLQNYRLTDATLYVTFEPCVMCAGAMIHSRIGRVVFGVRNSKRGAAGSLMNVLNYPGMNHCVEITEGILVDECAALLCDFYRMPRQVLNAQRKAQSSISPGGSSGGSSGSVTPGTSESPTPESSGGSSGGSAKNTITKALKLRIVRPYNSAEVEKIVADEKNNREKIALEKNKDKVKEACSKHLKVAAYCTTQVERNACLFCKARKLDDKFYQKLRGQFPDAVFWQEIGEIFRQLQRQAAEIYNQSLIELYYEIFIKGRGFANASSVEHYLSDVCYTRAAGLFKNAAIASGLRGKVKSNFRLKELKNMKSGLPTTKSDNFPIPLVKQKGGQYAGFEISSLNDDFIIKIPFGRWQVKKEIDKYRPWEKFDFEQVRKSPKPISLLLSTQRRKRNKGWSKDEGTEAEIRKVMNGDYQTSYIEVKRGSKTGEKSAWMLNLSIDVPKIDKGVDPSIIGGIDVGVKSPLVCAVNNAFSRYSISDNDLFRFNKKMFARRRILLRKNRHKRAGHGAKNKLKPISILTGKSERFRKKLIERWACEIADFFIKNKVGTVQMENLESMKRKEDSYFNIRLRGFWPYAEMQNKIEFKLKQYGIETRKVAPNNTSKTCSKCGHLNNYFNFEYRKKNKFPHFKCEKCNFKENADYNAALNISNPKLKSSKGEP

SEQ ID NO: 2109 - protein, 726 aa, synthetic construct
SEVEFSHEYWMRHALALAKRARDEREVPVGAVLVLNNRAIGEGWNRAIGLHDPTAHAEIMALRQGGLVMQNYRLTDATLYVTFEPCVMCAGAMIHSRIGRVVFGVRNSKRGAAGSLMNVLNCPGMNHCVEITEGILVDECAALLCDFYRMPRQVLNAQKKAQSSISSGGSSGGSSGSETPGASGSVTPKSSGGSSAGSTKDTITKTLKLRIVRPYNSAEVEKVVADEKNNREKIAIEKNKDMVKEACSKHLKVASYCTTQVERNACLFCKARKLDDKFYQKLRGQFPDAVFWQELGGIFRQLQKQAAEIYNQSLIELYYEIFIKGKGFANASSAEHYLSDVCYTRAAELFKNAAIASGLRGKVKSNFRLKELKNMKSGLPTTKSDNFPIPLVKQKGGKYTGFEISSHNDDFIIKIPFGRWQVKKEIDKYRPWEKFDFEQVRKSPKPISLLLSTQRRKRNKGWSKDEGTEAEIRKVMNGDYQTSYIEVKRGSKIGEKSAWMLNLSIDVPKIDKGVDPSIIGGIDVGVKSPLVCAINNAFSRYSISDNDLFHFNKKMFARRRILLKKSKHRRAGHGAKNKLKPITILTEKSKRFRKKLIERWACEIADFFIKNKVGTVQMENLESMKRKEDSYFNTRLRGFWPYAEMQNKIEFKLKQYGIEIRKVAPNNTSKTCSKCGHLNNYFNFEYRRKNKFPHFKCEKCNFKENADYNAALNISNPKLMSTKEEP

SEQ ID NO: 2110 - protein, 726 aa, synthetic construct
SEVEFSHEYWMRHALTLAKRARDEREVPVGAVLVLNNRVIGEGWNRAIGLHDPTAHAEIMALRQGGLVMQNYRLIDATLYVTFEPCVMCAGAMVHSRIGRVVFGVRNSKHGAAGSLVNVLDYPGMNHRVEITEGILADECAALLCDFYRMPRQVFNAQKKARPNINSGGSSGGRSGSVTPGTSESATPESSGGGFGGSVKNTITKTLQLRIVRPYNSAEVEKIVADEKNNREKIALEKNKDKVQEACSKHLKVASYCTTQVERNACLFCKARKLDDKFYQKLRGQFPDAVFWQELGEIFRQLQKQAAEIYNQSLIELYYEIFIKGKGPANASSVEHYLSDVCYTRAAELFKNAAIASGLRGKVKSNFKLKELKSMKSGLPSTKSDNFPIPLVKQKGGQYTGFEIRGHNDDLIIKIPFGRWQVKKEIDKYRPWEKFDFEQVRKSPKPISLLLSTQRRKRNKGWSKDEGTEAEIRKVMNGDYQTSYIEVKRGSKIGEKSAWMLNLSIDVPKIDKGVDPSIIGGIDVGVKSPLVCAINNAFSRYSVSDNDLFHFNKKMFARRRILLKKNRHKRAGHGAKNKLKPITILTEKSVRYRKKLIERWACEIADFFIKNKVGTVQMENLESMKGKEDSYFNIRLRGFWPYAEMQNKIEFKLKQYGIEIRKVAPNNTSKTCSKCGHLNNYFNFEYRKKNKFPHFKCEKCHFKEDADYNAALNISNPKLRCTKEEP

SEQ ID NO: 2111 - protein, 726 aa, synthetic construct
SEVEFSHEYWMRHALTLAKRARDEREVPVGAVLVLNNRVIGEGWNRAIGLHDPTAHAEIMALRQGGLVMQNYRLVDATLYVTFEPCVLCAGAMVHSRIGRVVFGVRNSKRGAAGSLMNVLNYPGMNHRVEITEGILADECAALLCDFYRMPRQVFNAQKKAQSSINSGGSSGGSSGSETPGTSESATPESSGGSSGGSAKNTITKTLKLRVVRPYNSAEVEKIVADEKNNREKIALEKNKDKVKEACSKHLKVAAYCTSQVERNACLFCKARKLDDRFYQKLRGQFPDAVFWQEVGEIFRQLQKQAAEIYNQSLIELYYEIFIKGKGFANASSVEHYLSDVCYTRAAELFKNAAIASGLRGKVKSNFRLKELKNMKSGLPTTKSDNFPIPLVKQKGGQYTGFEISSHNDDFIIKIPFGRWQVKKEIDKYRPWEKFDFEQVRKNPKPISLLLSTQRRKRNKGWSKDEGTEAEIRKVMNGDYQTSYIEVKRGSKIGEKSAWMLNLSIDVPKIDKGVDPSIIGGIDVGVKSPLVCAINNAFGRYSISDNDLFHFNKKMFARRRILLKKNRHKRAGHGAKNKLKPISILTEKSKRFRKKLIERWACEIADFFIKNKVGTVQMENLESMKRKEDSYFNIRLRGFWPYAEMQNKIEFKLKQYGIEIRKVAPNNTSKTCSKCGHLNSYFNFEYRKKNKFPHFKCEKCNFKENADYNAALNISNPKLKSTKGEP

SEQ ID NO: 2112 - protein, 726 aa, synthetic construct
SEVEFSHEYWMRHALTLAKRARDEHEVPVGAVLVLNNRVIGEGWNRAIGLHDPTAHAEIMALRQGGLVMQNYRLADATLYVTFEPCVMCAGAMIHSRIGRVVFGVRNSKRGAAGSLMNVLNYPGMNHCVEITEGILVDECAALLCDFYRMPRQVLNAQKKAQPNINPGGSSGGSGGSETPGTSGSATPKSSGGSSGGSAKNTVTKTLKLRIVRPYNSAEVEKIVADEKNNREKIALEKNKDKVKEACSKHLKVAAYCTTQVERNACLFCKARKLDDKFYQKLRGQFPDAVFWQEIGELFRQLQKQAAEIYNQSLVELYYEIFIKGKGFANASSVEHYLSDVCYTRAAELFKNAAIASGLRGKVKSNFRLKELKNMKSGLPTTKSDNFPIPLVKQKGGQYTGFEISSHNDDLIIKIPFGRWRVKREIDKYRPWEKFDFEQVRKSPKPISLLLSTQRRKRNKGWSKDEGTEAEIRKVMNGDYQTSYIEVKRGSKTGEKSAWMLNLSIDVPKIDKGVDPSIIGGIDVGVKSPLVCAINNAFSRYSISDNDLFRFNKKMFARRRILLKKNRHRRAGHGAKNKLKPISILTEKSERFRKKLIERWACEIADFFIRNKVGTVQMENLEGMKRKEDSYFNIRLRGFWPYAEMQDKIEFKLKQYGIEIRKVAPNNTSKTCSRCGHLNNYFNFEYRRKNKFPHFKCEKCNFKENADYNAALNISNPKLRSTKEEP

SEQ ID NO: 2113 - protein, 726 aa, synthetic construct
SEVEFSHEYWMRHALTLAKRARDEREVPVGAVLVLNNRVIGEGWNRAIGLHDPTAHAEIMALRQGGLVLQNYRLVDATLYVTFEPCVLCAGAMVHSRIGRVVFGARNSKRGAAGSLMNILNYPGMNHRVEITEGILADECAALLCDFYRMPRQVFNAQKKAQSSINSGGSSGGSSGSETPSTSESATPESSGGSSGGSAKNTITKTLQLRIVRPYNSAEVEKIVTDEKNNREKIALEKNRDKVKEACSKHLKMASYCTTQVERNACLFCKARKLDDKFYQKLRGQFPDAVFWQEIGEIFRQLQKQAAEIYNQSLIELYYEIFIKGKGFANASSVEHYLSDVCYTRAAELFKNAAIASGLRGKVKSNFRLKELKNMKSGLPTTKSDNFPIPLVKQKGGQYTGFEISSHNDDFIIKIPFGRWQVKKEIDKYRPWEKFDFEQVRKSPKPISLLLSTQRRKRNKGWSKDEGTEAEIKKVMNGDYQISYIEVKRGTKIGEKSAWMLNLSVDVPKIDKGVDPSIIGGIDVGVKSPLVCAINNAFSRYSISDNDLFHFNKKMFARRRILLKKNGHKRAGHGTKNKLKPITIMTEKSKRFRRKLIERWACEIADFFIKNKVGTVQMENLESMKRKEDSYFNIRLRGFWPYAELQNKIEFKLKQYGIVVRKVAPNNTSKTCSKCGHLNNYFNFEYRKKNKFPHFKCEKCNFKENADYNAALNISNPKLKSTKGEP

SEQ ID NO: 2114 - protein, 726 aa, synthetic construct
SEVEFSHEYWMRHALTLAKRARDEREVPVGAVLVLNNRVIGEGWNRAIGLHDPTAHAEIMALRQGGLVMQNYRLTDATLYVTFEPCVMCAGAMIHSRIGRVVFGVRNSKRGAAGSLMNVLNYPDMNHCVEITEGILVDECAALLCDFYRMPRQVLNAQKKAQSSISSGGSSGGSSGSETPGASESATPKSSGGSSAGSTKNTITKTLKLRIVRPYNSAEVEKIVADEKNNREKTALERNKDKVKEACSKHLKMAAYCTTQVERNACLFCKARKLDDKFYQKLRGQFPDAVFWQEVGEIFRQLQKQAAEIYNQSLIELYYEIFIKGKGFANASSVEHYLSDVCYTRAAELFKNAAIASGLRGKVKSNFRLKELKNMKSGLPTTKSDNFPIPLVRQKGGQYTGFEVSSHNDDFIIKIPFGRWQVKKEIDKYRPWEKFDFEQVRKSPRPISLLLSTQRRKRNKGWSKDEGTEAEIRKVMNGDYQTSYIEVKRGSKIGEKSAWMLNLSIDVPKIDKGVDPSIIGGIDVGVKSPLVCAIDNAFSRYSISDNDLYHFNKKMFAKRRILLKKNRHKRAGHGAKNKLKPISILTEKSERFRKKLIERWACEIADFFIKNKVGTVQMENLESMKRREDSYFNTRLRGFWPYAEMQNKIEFKLKQYGIEIRKVVPNNTSKTCSKCGHLNNYFNFEYRKKNKFPHFKCEKCNFKENADYNAALNISNPKLKSTKGEP

SEQ ID NO: 2115 - protein, 726 aa, synthetic construct
SEVEFSHEYWMRHALTLAKRARDEREVPVGAILVLNNRVIGEGWNRAIGLHDPTAHAEIMALRQGGLVMQNYRLIDATLYVTFEPCVMCAGAMIHSRIGRVVFGVRNSKHGAAGSLVNVLNYPGMNHRVEITEGILADECAALLCDFYRMPRQVFNARKKAQSSINSGGSSGGSSGSETPGTSESATPKSSGGSSGGSAKNTITKALKLRIVRPYNSAEVEKIVADEKNNRERIALEKNKDKVKEACSKHLKVAAYCTTQVERNACLFCKARKLDDKFYQKLRGQFPDAVFWQEIGEIFRQLQKQAAEIYNQSLIELYYEIFIKGRGFANASSVEHYLSDVCYTRAAELFKNAAIASGLRGKVKSNFRLRELKNMKSGLPTTKSDNFPIPLVKQKGGQYTGFEISNHNDDFIIKIPFGRWQVKKEIDKYRPWEKFDFEQVRKSPKPISLLLSTQRRKRNKGWSKDEGTEAEIRKVMNGGYQTSYIEVKRGSKTGEKSAWMLNLSIDVPKIDKGVDPSIIGGIDVGVKSPLVCAINNAFSRYSISDNDLFHFNKKMFARRRILLKKNRHKRAGHGAKNKLKPLTILTGKSKRFRKKLIERWACEIAGFFIKNKVGTVQMENLESMKRREDSYFNIRLRGFWPYAEMQNKIEFKLKQYGIEIRKVAPNNTSKTCSRCGHLNNYFNFEYRKRNKFPHFKCEKCNFKENADYNAALNISNPKLKSPKEEP

SEQ ID NO: 2116 - protein, 726 aa, synthetic construct
SEVEFSHEYWMRHALTLAKRARDEREVPVGAVLVLNNRVIGEGWNRAIGLHDPTAHAEIMALRQGGLVMQNYRLTDATLYVTFEPCVMCAGAMIHSRIGRVVFGVRNSKRGAAGSLMNVLNYPGMNHCVEITEGILVDECAALLCDFYRMPRQVLNAQKKAQSSINPGGSSGGSSGSETPGTSESPTPESPGGSSGGSAKNTITKTLKLRIVRPYNSAEVEKIVADEKNNREKIALEKNKDKVKEACSKHLKVAAYCTTQVERSACLFCKARRLDDKFYQKLRGQFPDAVFWQEIGEIFRQLQKQAAEIYNQSLIELYYEIFIKGKGFANASSVEHYLSDVCYTRAAELFKNAAIASGLRNKIKSNFRLKELRNMKSGLPTTKSDNFPIPLVRQKGGQYTGFEISSHNDDFIIKIPFGRWLVKKEIDKYRPWEKFDFEQVRKSPKPISLLLSTQRRKRNKGWSKDEGTEAEIRKVMNGDYQTSYIEVKRGSKIGEKSAWMLSLSIDVPKIDKGVDPRIIGGIDVGVKSPLVCAINNVLSRYSISDNDLFHFNKKMFARRRILLKKNRHRRAGHGAKNKLKPISILTEKSKRFRKKLIERWACEIADFFIKNKVGTVQMENLESMKRKEDSYFNIRLRGFWPYAEMQNKIEFKLRQYGIEIRKVAPNNTSKTCSKCGHLNSYFNFEYRKKYKFPYFKCAKCNFKENADYNAALNISNPKLKSTKEEP

SEQ ID NO: 2117 - protein, 726 aa, synthetic construct
SEVEFSHEYWMRHALTLAKRARDEREVPVGAILVLNNRVIGEGWNRTIGLHDPTAHAEIMALRQGGLVMQNYRLIDATLYVTFEPCVMCAGAMIHSRIGRVVFGIRNSKRGAAGSLMNVLNYPGMNHRVEIMEGILTDECAALLCDFYRMPRQVLNAQKKARSSTSSGGSSGSSRGSETPGTSESAAPGSSGGNSGGSAKNTITKTLRLRIVRPYNSTEVEKIVADEKNNREKIALEKNKDKVKEACSKHLKVASYCTTQVERNACLFCKARKLDDKFYQKLRGQFPDAVFWQELGEIFRQLQKQAAEIYNQSLIELYYEIFIKGKGFANASSVEHYLSDVCYTRAAELFKNAAIASGLRSKVRSNFRLKELKNMKSGLPTTKSDNFPIPLVKQKGGQYTGFEISSHNSDFIIKIPFGRWQVKEEIDKYRPWEKFDFEQVRKSPKPISLLLSTQRRKKNRGWSKDEGTEAEIRRVMNGDYQTSYIEVKRGSKIGEKSAWMLNLSIDVPKIDKGVNPSIIGGIDVGVKSPLVCAINNSSSRYSICDNDLFRFNKKMFARRRILLKKNRHKRAGHGAKNKLKPITILTERSKRFRKKLIERWACEIADFFIKNKVGTVQMENLEGMKRKEDSYFNIRLRGFWPYAEMQSKIEFKLKQYGIKIRKVAPNNTSKTCSKCGHLNNYFNFEFRKKNKFPHFRCEKCNFKENADYNAALNISNPRLKSTKEEP

SEQ ID NO: 2118 - protein, 726 aa, synthetic construct
SEVEFSHEYWMRHALTLAKRARDEREVPVGAVLVLNNRVIGEGWNRTTGLHDPTAHAEIMALRQGGLVMQNHRLVDATLYVTFEPCVMCAGAMIHSRIGRVVFGVRNSKRGAAGSLMNVLNYPGMNHRVEITEGILANECAALLCDFYRMPRQVFNARKKAQSSINPGGSSGGSSGSETPGTSESATPESSGGSSGGSAKNTITKTLKLRIVRPYNSAEVEKIVADEKNNREKIALEKNKDKVKEACSKHLKVAAYCTTQVERNACLFCKARKLDDKFYQKLRGQFPDAVFWQEIGEIFRQLQKQAAEIYNQGLIELYYEIFIKGKGFANASSVEHYLSDVCYTRAAELFKNAAIASGLRGKVKSNFRLKELKNMKSGLPTTKSDNFPIPLVKQKGGQYTGFEISSHNDDFIIKIPFGRWQAKEEIDKYRPWEKFDFEQVRKSPKPISLLLSTQRRKKNKGWSKDEGTEAEIRRVMNGDYQTSYIEVKRGSKIGEKSAWMLNLSIDVPKIDKGVDPSIIGGIDVGVKSPLVCAINNAFSRYSISDNDLFRFNKKMFARRRILLKKNRHKRAGHGAKNKLKPITILTEKSGRFRKKLIERWACEIADFFIKNKVGTVQMENLGSMKRKGDSYFNIRLRGFWPYAEMQNKIELKLKQYGIKIRKVAPNNTSKTCSKCGHLNDYFNFEYRKKNKFPHFKCEKCNFKEDADYNAALNISNPKLKSTREEP

SEQ ID NO: 2119 - protein, 726 aa, synthetic construct
SEVEFSHEYWMRHALTLAKRARDEREVPVGAVLVLNNRVIGEGWNRTTGLHDPTAHAEIMALRQGGLVMQNHRLVDATLYVTFEPCVMCAGAMIHSRIGRVVFGVRNSKRGAAGSLTNVLNYPGMNHRVEITEGILVDECAALLCDFYRMPRQVFNAQRKAQPTINSGGSSGGSSGSETPGTSESPTPESPGGSSGGSAKNTITKTLKLRIVRPYNSAEVEKIVADEKNNREKIALEKNKDKVKEACSKHLKVAAYCTTQVERNACLFCKARKLDDKFYQKLRGQFPDAVFWQEIGEIFRQLQKQAAEIYNQSLIELYYEIFIKGRGFANASSVEHYLSDVCYTRAAELFKNAAIASGLRGKVKSNFRLKELKNMKSGLPTTKSDNFPIPLVKQKGGQYTGFEISSHNDDFIIKIPFGRWQVKKEIDKYRPWEKFDFGQVRKSPKPISLLLSTQRRKGNKGWSKDEGTEAEIRKVMNGDYQTSYIEVKRGSKIGEKSAWMLNLSIDVPKIDKGVDPSIIGGIDVGVKSPLVCAINNAFSRYSISDNDLFHFNKKMFARRRILLKKTRHKRAGHGAKNKLKPISILTEKSERFRKKLIERWACEIADFFIKNKVGTVQMENLESMKRREDSYFNIRLRGFWPYAKMQNKIEFKLKQYGIEIRKVAPNNTSKTCSKCGHLNNYFNFEYRKKNKFPHFKCEKCNFKENADYNAALNISNPKLKSTKEEH

SEQ ID NO: 2120 - protein, 726 aa, synthetic construct
SEVEFSHEYWMRHALTLAKRARDEREVPVGAVLVLNNRVIGEGWNRAIGLHDPTAHAEIMALRQGGLVMQNYRLTDATLYVTFEPCVMCAGAMIHSRIGRVVFGVRNSKRGAAGSLMNVLNYPGMNHCVEITEGILVDECAALLCDFYRMPRQVLNAQKKAQSSISSGGLSGGSSGSETPGASGSATPKSSGGSSGGSAKNTITKALKLRIVRPYNSAEVEKIVADEKNNRERIALEKNKDKVKEACSKHLKVAAYCTTQVERNACLFCKARKLDDKFYQKLRGQFPDAVFWQELGEIFRQLQKQAAEIYNQSLIELYYEIFIKGKGFANASSVEHYLSDVCYTRAAELFKNAAIASGLRGKVKSNFRLKELRNMKSGLPTTKSDNFPIPLVKQKGGQCTGFEISNHNSDFIIKIPFGRWQVKKEIDKYRPWEKFNFEQVRKSPKPISLLLSTQRRKRNKGWSEDEGTEAEIRKVMNGDYQTSYIEVKRGSKIGEKSAWMLSLSIDVPKIDKGVDPSIIGGIDVGVKSPLVCAINNAFSRYSISDNDLFHFNKKMFARRRILLKKNRHKRAGHGAKNKLKPITILTEKSVRFRKKLIERWACEIADFFVKNKVGTVQMENLESMKRKEDSYFNIRLRGFWPYAEMQNKIEFKLKQYGIVVRKVAPNNTSKTCSQCGHLNNYFNFEYRKKSKFPYFKCEKCNFKENADYNAALNISNPQLKGTKGEP

SEQ ID NO: 2121 - protein, 726 aa, synthetic construct
SEVEFSHEYWMRHALTLAKRARDEREVPVGAILVLNNRVIGVGWNRAIGLHDPTAHAEIMALRQGGLVMQNYRLIDATLYVTFEPCIMCAGAMIHSRIGRVVFGVRNSKRGAAGSLMNVLNYPGMNHRVEITEGVLADECAALLCDFYRMPRQVLNAQKKAQSSINSGGSSGGSSGSETPGTSESPTPESSGGSSGGSAKNTITKTLKLRIVRPYNSAEVEKIVADEKNNREKIALEKNKDKVKEACSKHLKVAAYCTTQVERNACLFCKARRLDDKFYQKLRGQFPDAVFWQEIGEIFRQLQKQAAEIYNQSLIELYYEIFIKGKGIANASSVEHYLSDVCYTRAAELFKNAAIASGLRNKVKSNFRLKELRSMKSGLPTTKSDNFPIPLVRQKGGQYTGFGISNHNGDFIIKIPFGRWQVKKEINKHRPWEKFDFEQVRKSPKPISLLLSTQRRKRNKGWSKDEGTEAEIRKVMNGDYQTSYIEVKRGSKIGEKGAWMLNLSIDVPKIDKGVDPSIIGGIDVGVKSPLVCAINNALSRYSISDNDLFHFNKKMFARRRILLRKNRHKRAGHGARNKLKPITVLTEKSERFRRKLIERWACEIANFFIKNKVGTVQMENLESMKRREDSYFNIRLRGFWPYAEMQNKIEFKLKQYGIEIRKVAPNNTSKTCSKCGHLNNYFNFEFRKKNKFPHFKCEKCNFKEDADYNAALNISNPKLKSTKEEP

SEQ ID NO: 2122 - protein, 726 aa, synthetic construct
SEVEFSHEYWMRHALTLAKRARDEREVPVGAILVLNNRVIGEGWNRAIGLHDPTAHAEIMALRQGGLVMQNYRLTDATLYATFEPCVMCAGAMIHSRIGRVVFGVRNSKHGAAGSLMNVLNYPGMNHRVEITEGILADECAGLLCDFYRMPRQVFSARKKAQSSINPGGSSGDSSGGKAPGTSESATLESSGGSSGDSAKNSITKTLKLRIVRPYNSAEVEKIVADEKNNREKIALEKNKGKVEEACSKHLKVATYCTTQVERNACLFCKARKLDDKFYQKLRGQFPDAVFWQELGEIFRQLQKQAAEIYNQSLIELYYEIFIKGKGFANASSVEHYLSDVCYTRAAELFKNAAIASGLRGKVKSNFRLKELKNMKSGLPATKSDNFPIPLVKQKGGQYTGFEISSHNDDFIIKIPFGRWQAKKEIDRYRPWEKFDFEQVRKSPKPISLLLSTRRRKRNKGWSKDEGTEAEIRRVMNGDYQTSYIEVKRGSKIGEKSAWMLSLSIDVPKIDKGVDPRIIGGIDVGVKSPLVCAINNVLSRYSISDNDLFHFNKKMFARRRILLKKNGHKRAGHGAKNKLKPITIMTEKSKRFRKKLIERWACEIADFFIKNKVGTVQMENLESMKRKEDSYFNIRLRGFWPYAEMQNKIEFKLKQYGIVVRKVAPNNTSKTCSQCGHLNNYFNFEYRKKNKFPYFKCEKCNFKENADYNAALNISNPQLKSTKGEP

SEQ ID NO: 2123 - protein, 726 aa, synthetic construct
SEVEFSHEYWMRHALTLAKRARDEREVPVGAVLVLNNRVIGEGWNRAIGLHDPTAHAEIMALRQGGLVMQNYRLIDATLYVTFEPCVMCAGAMIHSRIGRVVFGVRNSKHGAAGSLVNVLNYPGMNHRVEITEGTLADECAALLCDFYRMPRQVFNARKKAQSSINPSGSSGGSSGSVTPGTSESATPESSGGGFGGSAKNTITKTLQLRIVRPYNSAEVEKIVADEKNNREKIALEKNKDKVKEACSKHLKVASYCTTQVERNACLFCKARKLDDKFYQKLRGQFPDAVFWQELGEIFRQLQKQAAEIYNQSLIELYYEIFIKGKGLASASSVEHYLSDVCYTRAAELFKNAAIASGLRGKVKSNFRLKELKNMKSGLPTTKSDNFPIPLVRQKGGQYTGFEISSHNDDFIIKIPFGRWQVKKEIDKYRPWEKFDFEQVRKSPKPISLLLSTQRRKRNKGWSKDEGTEAEIRKVMNGDYQTSYIEVRRGSKIGEKNAWMLSLSIDVPKIDKGVDPSIIGGIDVGVKSPLVCAINNAFSRYSISDNDLFRFNKKMFARRRILLKKNRHKRAGHGAKNKLRPISILTGKSERFRKKLIERWACEIADFFIKNKVGTVQMENLESMKRKEDSYFNIRLRGFWPYAEMQNKIEFKLKQYGIEIRKVAPNNTSKTCSKCGHLNNYFNFEYRKKSKFPHFKCEKCSFKEDADYNAALNISNPKLKSTKEEP

SEQ ID NO: 2124 - protein, 726 aa, synthetic construct
SEVEFSHEYWMRHALTLAKRACDEREVPVGAVLVLNNRVIGEGWNRAIGLHDPTAHAEIMALRQGGLVMQNYRLIDATLYVTFEPCVMCAGAMVHSRIGRVVFGVRNSKRGAAGSLMNVLDYPGMGHRVEITEGILADECAALLCDFYCMPRQVFNAQKRAQSSINSGGSSGGSSGSKTPGTSESATPGSSGGGSSGSAKNTITKTLQLRIVRPYNSAEVERILADEKDNREKIALERNKDKVKEACSKHLKVAAYCTTQVERNACLFCRARKLDDKFYQKLRGQFPDAVFWQEIGEIFRQLQKQAAEIYNQSLIELYYEIFIKGKGSANASSVEHYLSDVCYTRAAELFKNAAIASGLRGKVKSNFRLKELKNMKSGLPTTKSDNFPIPLVKQKGGQYTGFEISSHNDDFIIKIPFGRWQVKKETNKYRPWEKFDFEQVRKSPKPISLLLSTQRRMRNKGWSKDEGTEAEIRKVMNGDYQTSYIEVKRGSKIGEKSAWMLNLSIDVPKIDKGVDPSIIGGIDVGVKSPLVCAINNALSRYSISDNDLFHFNKKMFARRRILLKKNRHKRAGHGARNKLKPITVLTEKSERFRKKLIERWACEIANFFIKNKVGTVQMENLESMKRKEDSYFNIRLRGFWPYAEMQNKIEFKLKQYGIEIRKVAPNNTSKTCSKCGHLNNYFNFEYRKTNKFPYFKCEKCNFKEDADYNAALNISNPKLKSTKEEP

SEQ ID NO: 2125 - protein, 726 aa, synthetic construct
SEDEFSHEYWMRHALTLAKRARDGREVPVGAVLVLNNRVIGEGWNRAIGLHDPTAHAEIMALRQGGLVMQNYRLIDATLYVTFEPCVMCAGAMVHSRIGRVVFGVRNSKRGAAGSLMNVLDYPGMGHRVEITEGILADECAALLCDFYCMPRQVFNAQKRAQSSISPGGSSGGSSGSETPGASGSVTPKSSGGSSAGSTKDTITKTLKLRIVRPYNSAEVEKIVADEKNNREKIALEKNKDKVKEACSKHLKVAAYCTTQVERNACLFCKARRLDDKFYQKLRGQFPDAVFWQEIGEIFRQLQKQAAEVYNQSLVELYYEILIKGKGIANASSVEHYLSDVCYTRAAELFKNAAIASGLRNKIKSNFRLKELKNMKSGLPTTKSDNFPIPLVKQKGGQYTGFEISSHNDDFIIKIPFGRWQVKKEIDKYRPWEKFDFEQVRKSPKPISLLLSTQRRKRNKGWSKDEGTEAEIRKVMNGDYQTSYIEVKRGSKIGEKSAWMLNLSIDVPKIDKGVDPSIIGGIDVGVKSPLVCAINNAFSRYSISDNDLFRFNKKMFARRRILLRKNRHKRAGHGAKNKLKPITILTEKSERFRKKLIEKWACEIADFFIKNKVGTVQMENLESMKRKEDSYFNIRLRGFWPYAEMQNKIEFKLKQYGIEIRKVAPNNTSKTCSKCGHLNNYFNFEYRKKNKFPYFKCEKCNFKENADYNAALNISNPKLKSTKEEP

SEQ ID NO: 2126 - protein, 726 aa, synthetic construct
SEVEFSHEYWMRHALMLAKRARDEREVPVGAVLVLNNRVIGEGWNRAIGLHDPTAHAEIMALRQGGLAMQNYRLVDATLYVTFEPCVLCAGAMVHSRIGRVVFGVRNSKRGAAGSLMNVLNHPGMNHRVEITGGILADECAALLCDFYRMPRQVFNARKKARSNINSGGSSGGSSGSETPGTSESATPESSGGSSGGSAKNTITKTLTLRIVRPYNSAEVEKIVADEKNNRERIALEKNKDKVKEACSKHLKVAAYCTTQVERNACLFCKARKLDDRFYQKLRGQFPDAVFWQETGEILRQLQRQAAEIYNQSLIELYYEIFIKGKGFANASSVEHYLSDVCYTRAAELFKNAAIASGLRGKVKGNFRLKELKNMKSGLPTTKSDNFPIPLVKQKGGQYTGFEISSHNDDFIIKIPFGRWQAKKEIDKYRPWEKFDFEQVRKSAKPISLLLSTQRRKRNKGWSKDEGTEAEIRKVMNGDYQTSYIEVKRGSKIGEKSAWMLNLSIDVPKIDKGVDPSIIGGIDVGVKSPLVCAINNAFSRYSISDNDLFHFNKKMFARRRILLKKNRHKRAGHGAKNKLKPISILTEKSKRFRKKLIERWACEIADFFIKNKVGTVQMENLESMKRKEDSYFNIRLRGLWPYAEMQNKIEFKLKQYGIEIRKVAPNNTSKTCSKCGHLNNYFNFEYRRKNKFPHFKCEKCNFKEDADYNAALNISNPKLKSTKEEP

SEQ ID NO: 2127 - protein, 726 aa, synthetic construct
SEVEFSHEYWMRHALTLAKRARDEREVPVGAVLVLNNRVIGEGWNRAIGLHDPTAHAEIMALRQGGLVMQNYRLVDATLYVTFEPCVLCAGAMVHSRIGRVVFGVRNSKRGAAGSLMNVLNYPGMNHRVEITEGILADECAALLCDFYRMPRQVFNARKRARSNINSGGSSGGSSGSETLGTREGATPESSGGSSGGSAKNTITKTLKLRIVRPYNSAEVEKIVVDEKNNREKVALEKNKDKVKEACSEHLKVAAYCTTQVERSACLFCKARKLDDKFYQKLRGQFPDAVFWQEIGEIFRQLQKQAAEIYNQSLIELYYEIFIKGKGFANASSVEHYLSDVCYTRAAELFKNAAIASGLRGKVKSNFRLRELKNMKSGLPTTKSDNFPIPLVKQKGGQYTGFEISSHNDDFIIKIPFGRWQAKEEINKYRPWEKFDFEQVRKSPKPISLLLSTQKRKRNKGWSKDEGTEAEIRKVMNGDYQTSYIEVKRGSKTGEKSAWMLNLSIDVPKIDKGVDPSIIGGIDVGVKSPLVCAINNAFSRYSISDNDLFRFNKKMFARRRILLKRNRHKRAGHGAKNKLKPISTLTERSKRFRKKLIERWACEIADFFIKNKVGTVQMENLESMKRKEDSYFNIRLRGFWPYAEMQNKIEFKLKQYGIEIRKVAPNNTSKTCSKCGHLNNYFNFEYRKKNKFPHFKCEKCNFKENADYNAALNISNPKLKSTKKEP

SEQ ID NO: 2128 - protein, 726 aa, synthetic construct
SEVEFSHEYWMRHALTLAKRARDEREVPVGAVLVLNNRVIGEGWNRAIGLHDPTAHAEIMALRQGGLVMQNYRLIDATLYVTFEPCVMCAGAMVHSRIGRVVFGVRNSKRGAAGSLMNVLDYPGMNHRVEITEGILADECAALLCDFYRMPRQVFNAQRKAQSSINFGGSSGGSSGSGTPGTSESATPESSGGSSGGSAKNTITKTLKLRIVRPYNSAEVEKIVADEKNNREKIALEMNKDKVKEACSKHLKVASYCTTQVERNACPFCKARKLDDKFYQKLRGQFPDAVFWQELGEILRQLQKQAAEIYNQSLIELYYEIFIKGRGFANAGSVEHYLSDVCYTRAAGLFKNAAIASGLRGKVKSNFRLKELKNMKSGLPTTKSDNFPIPLVKQKGGQYAGFEISSHNDDFIIKIPFGRWQVKKEIDKYRPWEKFDFEQVRKSPKPISLLLSTQRRKRNKGWSKDEGTEAEIRKVMSGGYQTSYIEVKRGSKTGEKSAWMLNLSIDVPKIDRGVDPSIIGGIDVGVKSPLVCAINNALSRYSISDNDLFHFNKKMFARRRILLKKNRHKRAGHGAKNKLKPISVLTEKGERFRKKLIERWACEIADFFIKNKVGTVQMENLESMKRREDSYFNIRLRGFWPYAKMLNKIEFKLKQYGIKIRKVAPNNTSKTCSKCGHLNNYFNFEYRKKNKFPHFKCEKCNFKENADYNAALNISNPKLKSTKEEL

SEQ ID NO: 2129 - protein, 726 aa, synthetic construct
SEVEFSHEYWMRHALTLAKRARDEREVPVGAVLVLNNRVIGEGWNRAIGLHDPTAHAEIMALRQGGLVMQNYRLTGATLYVTFEPCVMCAGAMIHSRIGRVVFGVRNSKRGAAGSLMNVLNYPGMNHCVETTEGILVDECAALLCDFYRMPRQVLNAQKKAQSSISSGGSSGGSSCSETPGASESVTPKSSGGSSAGTTKNTITKTLKLRIVRPYNSAEVEKIVADEKNNREKIALERNRDKVKEACSEHLRVAAYCTTQVERNACLFCKARKLDDKFYQKLRGQFPDAVFWQELGEIFRQLQKQAAEIYNQSLIELYYEIFIKGKGFANASSVEHYLSDVCYTRAAELFKNAAIASGLRGKVKSNFRLKELKNMRSRLPTAKSDNFPIPLVKQKGGQYTGFEISSHNDDFIIKIPFGRWQVKKEIDKYRPWEKFDFEQVRKSPKPISLLLSTRRRKRNKGWSKDEGTEAEIRKVMNGDYQTSYIEVKRGSKIGEKSAWMLNLSIDVPKVDKGVDPSIIGGIDVGVKSPLVCAINNAFSRYSISDNDLFHFNKKMFARRRILLKKSRHKRAGHGAKNKLKPITILTEKSGRFRKKLIERWACEIADFFVKNKVGTVQMENLESMKGKEDSYFNIRLRGFWPYAEMQNKIEFKLKQYGIEIRKVAPNNTSKTCSKCGHLNSYFNFEYRKRNKFPHFKCEKCNFRENADYNAALNISNPKLRSTKEEP

SEQ ID NO: 2130 - protein, 726 aa, synthetic construct
SEVEFSHEYWMRHALTLAKRARDEREVPVGAILVLNNRVIGEGWNRAIGLHDPTAHAEIMALRQGGLVMQNYRLIDATLYVTFEPCVMCAGAMIHSRIGRVVFGVRNSKHGAAGSLMNVLNYPGMNHRVEITEGILADECAALLCDFYRMPRQVFNARKKAQSSISSGGSSGGSSGSETPGASGSVTPKSSVGSSAGSTKNTITKTLKLRIVRPYNSAEVEKIVADEKNNREKIALEKNKDKVKEACSKHLKVAAYCTTQVERNACLFCKARKLDDKFYQKLRGQFPDAVFWQEISEIFRQLQRQAAEIYNQSLIELYYEIFIKGKGLANASSVEHYLSDVCYTRAAELFKNAAIASGLRGKVKSNFKLKELKNMKSGLPTTKSDNFPIPLVKQKGGQYTGFEISSHNDDFIIKIPFGRWQVKREIDKYRPWEKFDFEQVRKSPKPISLLLSTQRRKRNKGWSKDEGTEAEIRKVMNGDYQTSYIEVKRGSKIGEKSAWMLSLSIDVPKIDKGVDPSIIGGIDVGVKSPLVCAINNAFCRYSISDNDLFHFNKKMFARRRILLKKSRHKRAGHGAKNKLKPISILTEKSKRFRKKLIERWACEIADFFIKNKVGTVQMENLESMKRKEDSYFNIRLRGFWPYAEMQNKIEFKLKQYGIEIRKVAPNNTSKTCSKCGHLNNYFNFEYRKKNKFPHFRCEKCSFKENADYNAALNISNPKLKSTREEP

SEQ ID NO: 2131 - protein, 726 aa, synthetic construct
SEVEFSHEYWMRHALTLAKRARDEREVPVGAVLVLNNRVIGAGWNRAIGLHDPTAHAEIMALRQGGLVTQNYRLINATLYVTFEPCVMCAGAMIHSRIGRVVFGVRNSKHGAAGSLVNVLNYPGMNHRVEITEGILADECAALLCDFYRMPRQVFNARKKAQSSINSGGSSGGSSGSETPGTSESATPKSSGGSSGGSAKNTITKTLQLRIVRPYNSAEVEKIVADEKNNREKIALEKNKDKVKEACSEHLKVAAYCTTQVERSACLFCKARKLDDKFYQKLRGQFPDAVFWQELGGIFRQLQKQAAEIYNQSLIELYYEIFIKGRGFANASSVEHYLSDVCYTRAAELFKNAAIASGLRGKVKSNFRLKELKNMKSGLPTTKSDNFPIPLVKQKGGQYTGFEISSHNDDFIIKIPFGRWQVKKEIDKYRPWEKFDFEQVRKSPKPISLLLSTQRRKRNKGWGKDEGTEAEIRKVMNGDYRTSYIEVKRGSKTGEKSAWMLNLSIDVPKIDKGVDPSIIGGIDVGVKSPLVCAVNNALSRYSIDDNDLFHFNKKMFARRRILLKKSKHKRAGHGAKNKLKPITILTEKSRRFRKKLIERWACEIADFFIKNKVGTVQMENLESMKRKEDSYFNIRLRGFWPYAEMQSKIEYKLKQYGIKIRKVAPNNTSKTCSKCGHLNNYFSFEYRKKNKFPHFKCEKCSFKEDADYNAALNISNPKLKSPKEEP

SEQ ID NO: 2132 - protein, 726 aa, synthetic construct
SEVEFSHEYWMRHALTLAKRARDEREVPVGAVLVLNNRVIGEGWNRAIGLHDPTAHAEIMALRQGGLVMQNCRLVDATLYVTFEPCVMCAGAMIHSRIGRVVFGVRNSKRGAAGSLMNVLNYPGMNHRVEITEGILADECAALLCDFYRMPRQVLSARRKAQSSISLGGSSGGSSGSETPGTSESATPESSGGSSGGSAKNTITKTLKLRIVRPYNSAEVEKIVADEKNNREKIALEKNKDKVKEACSEHLKVAAYCTTQVERNACLFCKARKLDDKFYLKLRGQFPDAVFWQEISEIFRQLQKQAAEIYNQSLIELYYEIFIKGKGFANASSVEHYLSDVCYTRAAELFKNAAIASGLRGKVKSNFRLKELKNMKSGLPTTKSDNFPIPLVKQKGGQYTGFEISSHNSDFIIRIPFGRWRVKEEIDKYRPWEKFDFEQVRKSPKPISLLLSTQRRKRNKGWSKDEGTEAEIRKLMNGDYQTSYIEVKRGSRIGEKNAWMLNLSIDVPKVDKGVDPSIIGGIDVGVRSPLVCAINNAFSRYSVSDNDLFRFNKKMFARRRILLKKNKHKRAGHGAKNKLKPISILTGKSERFRKKLIERWACEIADFFIKNKVGTVQMENLESMKRKEDSYFNIRLRGFWPYAEMQNKIEFKLKQYGIEIRKVAPNNTSKTCSKCGHLNNYFNFEYRKKNKFPRFKCEKCNFKENADYNAALNISNPKLKSTKEEP

SEQ ID NO: 2133 - protein, 726 aa, synthetic construct
SEVEFSHEYWMRHALTLAKRARDEREVPVGAILVLNNRVIGEGWNRAIGLHDPTAHAEIMALRQGGLVMQNYRLIDATLYVTFEPCVMCAGAMIHSRIGRVVFGVRNSKHGAAGSLVNVLNYPGMNHRVEITEGILADECAALLCDFYRMPRQVFNARKKAQSSINPSGSSGGSSGSVTPGTSESATPESSGGGFGGSAKNTITKTLQLRIVRPYNSAEVEKIVADEKNNREKIALEKNKDKVKEACSKHLKVASYCTTQVERNACLFCKARKLDDKFYQKLRGQFPDAVFWQELGEIFRQLQKQAAEIYNQSLIELYYVIFIKGKGLANASSVEHYLSDVCYTRAAELFKNAAIASGLRGKVKSNFKLKELKSMKSGLPSTKSDNFPIPLVKQRGGQYTGFEISSHNDDFIIKIPFGRWQAKKEIDKYRPWEKFDFEQVRKSPKPISLLLSTQRRKRNRGWSKDEGTEAEIRKVMNGDYQTSYIEVKRGSKIGEKSAWMLNLSIDVPKIDKGVDPSIIGGIDVGVKSPLVCAINNAFSRYSISDNDLFRFNKKMFARRRILLGKNRHKRAGHGVKNKLKPITILTEKSGRFRKKLIERWACEIADFFVKNKVGTVQMENLESMKRKEDSYFNIRLRGFWPYAEMQNKIEFKLKQYGIKVRKVAPNNTSKTCSKCGHLNNYFNFEYRKKNKFPHFKCERCNFKENADYNAALNISNPKLKSTKEEP

SEQ ID NO: 2134 - protein, 726 aa, synthetic construct
SEVEFSHEYWMRHALTLAKRARDEREVPVGAILVLNNRVIGEGWNRAIGLHDPTAHAEIMALRQGGLVMQNYRLIDATLYVTFEPCVMCAGAMIHSRIGRVVFGARNSKHGAAGSLVNVLNYPGMNHRVEITEGILADECAALLCDFYRMPRQVFNARKKAQSSINPSGSSGGSSGSVTPGTSESATPESSGGGFGGSAKNTITKTLQLRIVRPYNSAEVEKIVADEKNNREKIALEKNKDKVKEACGKHLKVASYCTTQVERNACLFCKARKLDDKFYQKLRGQFPDAVFWQELGEIFRQLQKQAAEIYNQSLIELYYEIFIKGKGLANASSVEHYLSDVCYTRAAELFKNAAIASGLRGKVKSNFKLKELKSMKSGLPSTKSDNFPIPLVKQRGGQYTGFEISSHNDDFIIKIPFGRWQAKKEIDKYRPWEKFDFEQVRKSPKPISLLLSTQRRKRNRGWSKDEGTEAEIRKVMNGDYQTSYIEVKRGSKIGEKSAWMLNLSIDVPKIDKGVDPSIIGGIDVGVKSPLVCAINNAFSRYSISDNDLYRFNKKMFARRRILLGKNRHKRAGHGVKNKLKPITILTEKSGRFRKKLIERWACEIADFFVKNKVGTVQMENLESMKRKEDSYFNIRLRGFWPYAEMQNKIEFKLKQYGIKVRKVAPNNTSKTCSKCGHLNNYFNFEYRKKNKFPHFKCEKCNFKENADYNAALNISNPKQMSTKEGP

SEQ ID NO: 2135 - protein, 726 aa, synthetic construct
SEVEFSHEYWMRHALTLAKRARDEREVPVGAILVLNNRVIGEGWNRAIGLHDPTAHAEIMALRQGALVMRNYRLVDATLYVTFEPCVMCAGAMIHSRIGRVVFGVRNNKHGAAGSLVNVLNYPGMNHRVEITEGILVDECAALLCDFYRMPRQVLNARKKAQSSINPGGSSGGSSGSETPGTSESATPESSGGSSGGSAKNTITKTLKLRIVRPYNSAEVEKIVADEKNNREKIALKKNKDKVREACSKHLKVAAYCTTQVERSACLFCKARRLDDKFYQKLKGQFPDAVFWQEIGEILRQLQKQAAEIYNQSLVELYYEIFIKGKGIANASSVEHYLSDVCYTRAAELFKNAAIASGLRGKVKSNFKLKELKSMKSGLPSTKSDNFPIPLVKQKGGQYTGFEIRGHNDDLIIKIPFGRWQAKKEIDKYRPWEKFDFEQVRKSPKPISLLLSTQGRKRNRGWSKDEGTEAEIRKVMNGDYQTSYIEVKRGSKIGEKSAWMLNLSIDVPKIDKGVDPSIVGGIDVGVKSPLVCAINNAFSRYSISDNDLFRFNKKMFARRRILLGKNRHKRAGHGVKNKLKPITILTEKSKRFRKKLIERWACEIADFFIKNKVGTVQMENLESMKKREDSYFNIRLRGFWPYAEMQNKIEFKLKQYGIEIRKVAPNNTSKTCSKCGHLNNYFNFEYRKKNKFPHFKCEKCNFKENADYNAALNISNPKLKSTKEEP

SEQ ID NO: 2136 - protein, 726 aa, synthetic construct
SEVEFSHEYWMRHALTLAKRARDEREVPVGAVLVLNNRVIGEGWNRAIGLHDPTAHAEIMALRQGGLVMQNYRLIDATLYVTFEPCVMCAGAMVHSRIGRVVFGVRNSKRGAAGSLMNVLDYPGMGHRVEITEGILADECAALLCDFYCMPRQVFNAQKRAQSSINPSGSSGGSSGSVTPGTSESATPESSGGGFGGSAKNTITKTLQLRIVRPYNSAEVEKIMADEKNNREKIALEKNKDKVKEACSKHLKVASYCTTQVERNACLFCKARKLDDKFYQKLRGQFPDAVFWQELGEIFRQLQKQAAEIYNQSLIELYYVIFIKGKGLANASSVEHYLSDVCYTRAAELFKNAAIASGLRGKVKSNFKLKELKSMKSGLPSTKSDNFPIPLVKQRGGQYTGFEISSHNDDFIIKIPFGRWQAKKEIDKYRPWEKFDFEQVRKSPKPISLLLSTQRRKRNRGWSKDEGTEAEIRKVMNGDYQTSYIEVKRGSKIGEKSAWMLNLSIDVPKIDKGVDPSIIGGIDVGVKSPLVCAINNAFSRYSISDNDLFRFNKKMFARRRILLGKNRHKRAGHGVKNKLKPITILTEKSGRFRKKLIERWACEIADFFIKNKVGTVQMENLESMKRREDSYFNIRLRGFWPYAEMQNKIEFKLKQYGIEIRKVAPNNTSKTCSKCGHLNNYFNFEYRKKNKFPHFKCEKCNFKENADYNAALNISNPKLKSTKEEP

SEQ ID NO: 2137 - protein, 726 aa, synthetic construct
SEVEFSHEYWMRHALTLAKRARDEREVPVGAILVLNNRVIGEGWNRAIGLHDPTAHAEIMALRQGGLVMQNYRLIDATLYVTFEPCVMCAGAMIHSRIGRVVFGVRNNRHGAAGSLVNVLDYPGMNHRVAITEGILADECAALLCDFYRMPRQVFNARKKAQSSISPGGSSGGSSGSETPGTSESATPESSGGGSSGSAKNTITKTLQLRIVRPYNSAEVEKIVADEKNNREKIALEKNKDKVKEACGKHLKVASYCTTQVERNACPFCKARKLDDKFYQKLRGQFPDAVFWQELGEILRQLQKQAAEIYNQSLIELYYEIFIKGRGFANAGSVEHYLSDVCYTRAAELFKNAAIASGLRGKVKSNFRLKELKNMKSGLPTTKSDNFPIPLVKQKGGQYTGFEISSHNGDFIIKIPFGRWQVKKEIDRYRPWEKFDFEQVRKSPKPISLLLSTQRRKRNKGWSKDEGTEAEIRKVMNGDYQTSYIEVKRGSKIGEKSTWMLNLSIDVPKIDKGVDPSIIGGIDVGVKSPLVCAINNAFSRYSICDNDLFRFNKKMFARRRILLKKNRLRRAGHGAKNKLKPITVLTKKSERFRKKLIERWVCEVADFFIKNKVGTVQMENLESMKRKEDSYFNIRLRGFWPYAEMQNKIEFKLKQYGIKIRRVAPNNTSKTCSKCGHLNNYFSFEYRKKNKFPHFKCEKCNFKEDADYNAALNISSPKLKSTKEEP

SEQ ID NO: 2138 - protein, 726 aa, synthetic construct
SEVEFSHEYWMRHALTLAKRARDEREVPVGAVLVLNNRVIGEGWNRAIGLHDPTAHAEIMALRQGGLVMRNHRLVDATLYVTFEPCVLCAGAMVHSRIGRVVFGVRNSKRGAAGSLMNVLNYPGMNHRVEITEGILADECAALLCDFYRMPRQVFNARKKARSNINSGGSSGGSSGSETLGTREGATRESSGGSSGGSAKNTITKTLKLRIVRPYNSAEVEKIVVDEKNNREKVALEKNKDKVKEACSEHLKVAAYCTTQVERSACLFCKARKLDDKFYQKLRGQFPDAVFWQELGEIFRQLQKQAAEIYNQSLIELYYEIFIKGKGLANASSVEHYLSDVCYTRAAELFKNAAIASGLRGKVKSNFKLKELKSMKSGLPSTKSDNFPIPLVKQKGGQYTGFEISNHNGDFIIKIPFGRWQVKKEINKHRPWEKFDFEQVRKSPKPISLLLSTQRRKGNKGWSKDEGTEAEIRRVMNGDYQTSYIEVKRGSKIGEKSAWMLNLSIDVPKIDKGVNPSIIGGIDVGVKSPLVCAINNAFSRYSISDNDLFRFNKKMFARRRILLRKNRHKRAGHGAKNKLKPISILTGKSERFRKKLIERWACEIADFFTKNKVGTVQMENLESMKRKEDSYFNIRLRGFWPYAEMQNKIEFKLKQYGIEIRKVAPNNTSKTCSKCGHLNNYFNFEYRKKNKFPHFKCEKCNFKENADYNAALNISNPKLKSTKEEP

SEQ ID NO: 2139 - protein, 726 aa, synthetic construct
SEVEFSHEYWMRHALTLAKRARDEREVPVGAILVLNNRVIGEGWNRAIGLHDPTAHAEIMALRQGGLVMQNYRLIDATLYVTFEPCVMCAGAMIHSRIGRVVFGVRNNKHGAAGSLVNVLDYPGMGHRVEITEGILADECAALLCDFYCMPRQVFNAQKRAQSSINSGGSSGGSSGSETPGTSESATPESSGGGSSGSAKNTITKTLQLRIVRPYNSAEVEKIVADEKNNREKIALEKNKDKVKEACSKHLKVASYCTTQVERNACPFCKARKLDDKFYQKLRGQFPDAVFWQELGEILRQLQKQAAEIYNQSLIELYYEIFIKGRGFANASSVEHYLSDVCYTRAAELFKNAAIASGLRGKVKSNFRLKELKNMKSGLPTTKSDNFPIPLVKQKGGQYTGFEISSHNDDFIIKIPFGRWQVKEEIDKYRPWEKFDFEQVRRNPKPISLLLSTQRRKRNKGWGKDEGTEAEIRKVMNGDYQTSYIEVKRGSKIGEKSAWMLSLSIDVPKIDKGVDPGIIGGIDVGVKSPLVCAINNASSRYSISDNDLFHFNKKMFARRRILLKKNGHKRAGHGAKNKLKPITIMTEKSKRFRKKLIERWACEIADFFIKNKVGTVQMENLESMKRKEDSYFNIRLRGFWPYAEMQNKIEFKLKQYGIVVRKVAPNNTSKTCSQCGHLNNYFNFEYRKKNKFPHFKCEKCNFKENADYNAALNISNPKLKSTKKEP

SEQ ID NO: 2140 - protein, 725 aa, synthetic construct
SEVEFSHEYWMRHALTLAKRARDEREVPVGAVLVLNNRVIGEGWNRAIGLHDPTAHAEIMALRQGGLVMQNYRLIDATLYVTFEPCVMCAGAMVHSRIGRVVFGVRNSKRGAAGSLMNVLDYPGMGHRVEITEGILADECAALLCDFYCMPRQVFNAQKRAQSSINPGGSSGGSSGSETPGTSESASPESSGGGSSGSAKNTITKTLQLRIVRPYNSAEVEKIVADEKNNREKIALEKNKDKVKEACSKHLKVASYCTTQVERNACPFCKARKLDDKFYQKLRGQFPDAVFWQELGEILRQLQKQAAEIYNQSLIELYYEIFIKGRGFANACSVEHYLSDVCYTRAAELFKNAAIASGLRGKVKSNFRLKELKNMKSGLPTTKSDNFPIPLVKQKGGQYTGFEISSHNDDFIIKIPFGRWQVKKEIDKYRPWEKFDFEQVRKNPKPISLLLSIQRRKRNKGWSKDEGTEAEIRKVMNGDYQTSYIEVKRGSKIGEKSAWMLNLSIDVPKIDKGVDPSIIGGIDVGVKSPLVCAINNAFSRYSISDNELFHFNKKMFARRRILLKKNRHKRAGHGAKNKLKPITILTEKSVRFRKKLIERWACEIADFFIKNKVGTVQMENLESMKGKEDSYFNIRLRGFWPYAEMQNKIEFKLKQYGIEIRKVAPNNTSKTCSKCGHLNNYFNFEYRKKNKFPHFKCEKCYFKEDADYNAALNISNPRLKSTKEP

SEQ ID NO: 2141 - protein, 726 aa, synthetic construct
SEVEFSHEYWMRHALTLAKRARDEREVPVGAVLVLNNRVIGEGWNRAIGLHDPTAHAEIMALRQGGLVMQNYRLVDATLYVTFEPCVLCAGAMVHSRIGRVVFGVRNSKRGAAGSLMNVLNYPGMNHRVEITEGVLADECAALLCDFYRMPRQVFNAQKKARSNINSGGSSGGSSGSEAPGTSESATPESSGGGFGGSAKNTITKTLQLRIVRPYNSAEVEKIVADEKNNREKIALEKNKGKVKEACSKHLKVATYCTAQVERNACLFCKARKLDDKFYRKLRGQFPDAVFWQELGEIFRQLQKQAAEIYNQSLIELYYEIFVKGKGFANASSVEHYLSDVCYTRAAELFKNAAIASGLRGKVKSNFRLKELKNMKSGLPTTKSDNFPIPLVKQKGGQYTGFEISSRNDDFIIKIPFGRWQVKKEIDKYRPWEKFDFEQVRKSPKPISLLLSTQRRKRNRGWGKDEGTEAEIKRVMNGDYQTSYIEVKRGSKIGEKSAWMLNLSIDVPKIDKGVDPRIIGGIDVGVKSPLVCAINNAFSRYSVSDNDLFHFNKKMFARRRILLKKNRHKRAGHGAKNKLKPITILTEKSVRFRKKLIERWACEIADFFIKNKVGTVQMENLESLKRKEDSYFNIRLRGFWPYAEMQNKIEFKLKQYGIKVRKVAPNNTSKTCSKCGHLNNYFSFEYRKKNKYPHFKCEKCNFKENADYNAALNISNPKLKSTKEEP

SEQ ID NO: 2142 - protein, 726 aa, synthetic construct
SEVEFSHEYWMRHALTLAKRARDEREVPVGAILVLNNRVIGEGWNRAVGLHDPTAHAEIMALRQGGLAMQNYRLTDATLYVTFEPCVMCAGAMIHSRIGRVVFGVRNSKRGAAGSLMNVLNYPGMNHCVEITEGILVDECAALLCDFYRMPRQVFNAQKKAQSTINSGGSSGGSNGSETPGTSESPTPESSGGSPGGSAKNTITKTLKLRIVRPYNSAEVEKIVADEKNNREKIALEKNKDKVKEACSKHLKVAAYCTTQVERNACLFCKARKLDDKFYQKLRGQFPDAVFWQEIGEIFRQLQKQAAEIYNQSLIELYYEIFIKGKGFANASSVEHYLSDVCYTRAAELFKNAAIASGLRGKVKSNFRLKELKNMKSGLPTTKSDNFPIPLVKQKGGQYTGFEISNHDGDFIIKIPFGRWQVKKEINKHRPWEKFDFEQVRKSPKPISLLLSTQRRKRNKGWSKDEGTEAEIRKVMNGDYQTSYIEVKRGSKIGEKSAWMLNLSIDVPKIDKGVDPSIIGGIDVGVKSPLVCAINNAFSRYSISDNDLFRFNKKMFARRRILLKKNRHKRAGHGAKNKLKPITILTEKSGRFRKKLIERWACEIADFFIKNKVGTVQMENLESMKRREDSYFNIRLRGFWPYAEMQNKIEFKLKQYGIEIRKVAPNNTSKTCSKCGHLNNYFNFEYRKKNKFPHFKCEKCSFKENADYNAALNISNPKLKSTKEEP

SEQ ID NO: 2143 - protein, 726 aa, synthetic construct; identical to SEQ ID NO: 684

SEQ ID NO: 2144 - protein, 726 aa, synthetic construct
SEVEFSHEYWMRHALTLAKRARDEREVPVGAILVLNNRVIGEGWNRAIGLHDPTAHAEIMALRQGGLVMQNYRLIDATLYVTFEPCVMCAGAMIHSRIGRVVFGVRNSKHGAAGSLVNVLNYPGMNHCVEITEGILMDECAALLCDFYRMPRQVLNAQRKAQSSISSGGSSGGSSGSETPDTSGSATPESSGGSSGSSAKNTITKTLKLRIVRPYNSAEVEKIVADEKNNRERIALEKNKDKVKEACSKHLKVAAYCTTQVERNACLFCKARKLDDKFYRKLRGQFPDAVFWQEIGEIFRQLQKQAAEIYNQSLIELYYEIFIKGKGFANASSVEHYLSDVCYTRAAELFKNAAIASGLRGKVKGNFRLKELKNMKSGLPTTKSDNFPIPLVRQKGGQYTGFEISSHNDDFIIKIPFGRWQVRKEIDKYRPWEKFDFEQVRKSPKPISLLLSTQRRKRNKGWSKDEGTEAEIRKVMNGDYQTSYIEVKRGSKTGEKSAWMLNLSIDVPKIDKGVDPSIIGGIDVGVKSPLVCAINNAFSRYSISDNDLFHFNKKVFARRRILLKKNRHKRAGHGAKNKLKPITILTEKSKRFRKKLIERWACEIADFFIKNKVGTVQMENLESMKRKEDSYFNIRLRGFWPYAEMQNKIEFKLEQYGIKIRKVAPNNTSRTCSKCGHLNNYFSFEYRKKNKFPHFKCEKCNFKEDADYNAALNISNPKLKGTKEEL

SEQ ID NO: 2145 - protein, 726 aa, synthetic construct
SEVEFSHEYWMRHALTLAKRARDEREVPVGAILVLNNRVIGEGWNRAIGLHDPTAHAEIMALRQGGLVMQNYRLIDATLYVTFEPCVMCAGAMIHSRIGRVVFGVRNSKHGAAGSLMNVLNYPGMNHRVEITEGVLADECAALLCDFYRMPRQVFSARKKAQSSINPGGSSGGSSGSKTPGTSESATPESSGGSSGGSAKNSITKTLKLRIVRPYNSAEVEKIVADEKNNREKIALEKNKGKVKEACSKHLKVATYCTTQVERNACLFCKARKLDDKFYQKLRGQFPDAVFWQEIGEIFRQLQKQAAEIYNQSLIELYYEIFIKGKGFANASSVEHYLSDVCYTRAAELFKNAAIASGLRNKIKSNFRLKELRNMKSGLPTTKSDNFPIPLVRQKGGQYTGFEISNHNGDFIIKIPFGRWQVKKEINKHRPWEKFDFEQVRKSPKPISLLLSTQRRKRNKGWSKDEGTEAEIRKVMNGDYQTSYIEVKRGSKIGEKSAWMLNLSIDVPKIDKGVDPSITGGIDVGVKSPLVCAINNALSRYSISDNDLFHFNKKMFARRRILLRKNRHKRAGHGARNKLKPVTVLTEKSERFRKKLIERWACEIANFFIKNKVGTVQMENLESMKRREDSYFNIRLRGFWPYAEMQNKIEFKLKQYGIEIRKVAPNNTSKTCSKCGHLNNYFNFEFRKKNKFPHFKCEKCNFKENADYNAALNISNPKLKSTKEEP

SEQ ID NO: 2146 - protein, 726 aa, synthetic construct
SEVEFSHEYWMRHALTLAKRARDEREVPVGAVLVLNNRAIGEGWNRAIGLHDPTAHAEIMALRQGGLVMQNYRLTDATLYVTFEPCVMCAGAMIHSRIGRVVFGVRNSKRGAAGSLMNVLNYPGMNHSVEITEGILVDECAALLCDFYRMPRQVLNAQKKAQSSISSGGSSGGSSGSETPGASGSVIPKSSGGSSAGSTKDTITKTLKLRIVRPYNSAEVEKVVADEKNNREKIAMEKNKDKVKEACSKHLKVAAYCTTQVERNACLFCRARKLDDKFYQKLRGQFPDAVFWQEIGEIFRQLQKQAAETYNQSLIELYYEIFIKGKGFANASSVEHYLSCVCYTRAAELFKNAAIASGLRGKVKSNFRLKELKNMKSGLPTTKSDNFPIPLVKQKGGQYAGFEISSHNDDFIIKIPFGRWQVKKEIDKYRPWEKFDFEQVRKSPKPISLLLSTQRRKRNKGWSKDEGTEAEIRKVMNGDYQTSYIEVKRGSKIGEKSAWMLNLSIDVPKIDKGVDPSIIGGIDVGVKSPLVCAINNAFSRYSISDNDLFRFNKKMFARRRILLGKNRHKRAGHGVKNKLKPITILTEKSGRFRKKLIERWACEIADFFVKNKVGTVQMENLESMKRKEDSYFNIRLRGFWPYAEMQNKIEFKLKQYGIKVRKVAPNNTSKTCSKCGHLNNYFSFEYRKKNKFPHFKCEKCNFKENADYNAALNISNPKLKSTKEEP

SEQ ID NO: 2147 - protein, 726 aa, synthetic construct
SEVEFSHEYWMRHALSLAKRARDEREVPVGAVLVLNNRVIGEGWNRAIGLHDPTAHAEIMALRQGGLVMQNYRLIDATLYATFEPCVMCAGAMIHSRIGRVVFGVRNNKHGAAGSLVNVLNYPGMNHRVEITEGILADECAALLCDFYRMPRQVFNAQKKAQSSISSGGPSGSSSCSETPGASESVTPKSSGGSSTGSTKNTITKTLKLRIVRPYNSAEVEKIVADEKNNREKIALEKNKDKVKEACSKHLKVAAYCTTRVDRNACLFCKARRLDDKFYQKLRGQFPDALFWQEIGEIFRQLQKQAAEVYNQSLVELYYEILIKGKGIANASSVEHYLSDVCYTRAAELFKNAAIASGLRNKIKSNFRLKELRNMKSGLPTTKSDNFPIPLVRQKGGQYTGFEISNYNGDFIIKIPFGRWQVKKEINKHRPWEKFDFEQVRKSPKPISLLLSTQRRKRNKGWSKDEGTEAEIRKVMNGDYQTSYIEVKRGSKTGEKSAWMLNLSIDVPKIDKGVDPSIIGGIDVGVKSPLVCAINNAFSRYSISDNDLFHFNKKMFARRRILLKKNRHKRAGHGAKNKLKPISILTEKSKRFRKKLIERWACEIADFFIKNKVGTVQMENLESMKRKEDSYFNIRLRGFWPYAEMQNKIEFKLKQYGIEIRKVAPNNTSRTCSKCGHLNNYFNFEYRRKNKFPHFKCEKCNFKEDADYNAALNISNPKLKNTKEEP

SEQ ID NO: 2148 - protein, 726 aa, synthetic construct
SEVEFSHEYWMRHALTLAKRARDGREVPVGAVLVLNNRVIGEGWNRAIGLHDPTAHAEVMALRQGGLVMQNYRLIDATLYVTFEPCAMCAGAMVHSRIGRVVFGVRNSKRGAAGSLMNVLNYPGMDHRVEITGGILADECAALLCDFYRMPRRVFDAQKKAQSSINPGGSSGGSSGSKTPGTSESATPESSGGSSAGSTKNTITKTLKLRIVRPYNSAEVEKIVADEKNNREKIALEKNKDKVQEACSKHLKVASYCTTQVERNACLFCKARKLDDKFYQKLRGQFPDAVFWQELGEIFRQLQKQAAEIYNQSLIELYYKIFIKGKGLANASNVEHYLSDVCYTRAAELFKNAAIASGLRGKVKGNFRLKELKNMKSGLPTTKSDNFPIPLVKQKGGQYTGFEISSHNDDFIIKIPFGRWQVKKEIDKYRPWEKFDFEQVRKSPKPISLLLSTQRRKRNKGWSKDEGTEAEIRKVMNGDYQTSYIEVKRGSKIGEKSAWMLNLSIDVPKIDKGVDPSIIGGIDVGVKSPLVCAINNAFSRYSISDNDLFHFNKKMFARRRILLKKNRHKRAGHGAKNKLKPISILTEKSKRFRKKLIERWACEIADFFIKNKVGTVQMENLESMKRKEDSYFNIRLRGFWPYAEMQNKIELKLKQYGIEIRKVAPNNTSKTCSKCGHLNNYFNFEYRRKNKFPHFKCEKCNFKEDADYNAALNISNPKLKSTKEGP

SEQ ID NO: 2149 - protein, 726 aa, synthetic construct
SEVEFSHEYWMRHALTLAKRARDGREVPVGAVLVLNNRVIGEGWNRVIGLHDPTAHAEIMALRQGGLVMQNYRLIDATLYVTFEPCVMCAGAMVHSRIGRVVFGVRNSKRGAAGSLMNVLDYPGMGHRVEITEGILADECAALLCDFYCMPRQVFNAQKRAQSSINSGGSSGGSSGSDTPGTSESATPESSGGGSSGSAKNTITKTLQLRIVRPYNSAEVEKIVADEKNNREKIALEKNKDKVREACSKHLKVASYCTTQVERNACPFCKARKLDDKFYQKLRGQFPDAVFWQELGEILRQLQKQAAEVYNQSLIELYYEIFVKGKGFANASSVEHYLSDVCYTRAAELFKNAAIASGLRGKVKSNFRLKELKNMKSGLPTTKSDNFPIPLVKQKGGQYTGFEISSHNDDFIIKIPFGRWQVKEEIDRYRPWEKFDFEQVRKSPKPISLLLSTQRRKRNKGWSKDEGTEAEIRKVMNGDYQTSYIEVRRGSKTGEKSAWMLNLSIDVPKIDKGVDPSIIGGIDVGVKSPLVCAINNAFSRYSISDNDLFRFNKKMFARRRILLKKNRHKRAGHGAKNKLKPISILTGKSERFRKKLIERWACEIADFFIKNKVGTVQMENLESMKRKEDSYFNIRLRGFWPYAEMQNKIEFRLKQYGIEIRKVAPNNTSKTCSKCGHLNNYFNFEYRKKNKFPHFKCEKCNFKENADYNAALNISNPKLKSTKEEP

SEQ ID NO: 2150 - protein, 726 aa, synthetic construct
SEVEFSHEYWMRHALTLAKRARDGREVPVGAVLVLNNRVIGEGWNRAIGLHDPTAHAEIMALRQGGLVMQNYRLIDATLYVTFEPCVMCAGAMIHSRIGRVVFGVRNNKHGAAGSLVNVLNYPGMNHRVEIMEGILADECAALLCDFYRMPRQVFNARKKAQSSISPGGSSGGSSGSETPGTSESATPKNSGGSSGGSAKNTITKALKLKIVRPYNSAEVEKIVADEKNNRERIALEKNKDKVKEACSKHLKVAAYCTTQVERNACLFCKARKLDDKFYQKLRGQFPDAVFWQEIGEIFRQLQKQAAEIYNQSLIELYYEIFIKGKGFANASSVEHYLSDVCYTRAAELFKNAAIASGLRGKVKSNFRLKELKNMRSGLPTTKSDNFPIPLVKQKGGQYAGFEISSHNGDFIIKIPFGRWQVKKEIDKYRPWEKFDFEQVRKSPKPISLLLSTRRRKRNKGWSKDEGTEAEIRKVMNGDYQTSYIEVKRGSKIGEKSAWMLNLSIDVPKIDKGVDPSIIGGIDVGVKSPLVCAINNAFGRYSISDNDLFHFNKKMFARRRILLKKNRHKRAGHGAKNKLKPISILTGKSERFRKKLIERWACEIADFFIKSKVGTVQMENLESMKRREDSYFNIRLRGFWPYAEMQNKIEFKLKQYGIEIRKVAPNNTSKTCSKCGHLNNYFNFEYRKKNKFPHFKCEKCNFKENADYNAALNISNPKLKSTKEEP

SEQ ID NO: 2151 - protein, 726 aa, synthetic construct; identical to SEQ ID NO: 684

SEQ ID NO: 2152 - protein, 726 aa, synthetic construct
SEVEFSHEYWMRHALTLAKRARDEREVPVGAVLVLNNRVIGEGWNRAIGLHDPTAHAEIMALRQGGLAMQNYRLVDATLYVTFEPCVLCAGAMVHSRIGRVVFGVRNSKRGAAGSLMNVLNHPGMNHRVEITEGILADECAALLCDFYRMPRQVFNARKKAQSSINPSGSSGGSSGSVTPGTSESATPESSGGGFGGSAKNTITKTLQLRIVRPYNSAEVEKIVADEKNNREKIALEKNKDKVKEACSKHLKVASYCTTQVERNACLFCKARKLDDKFYQKLRGQFPDAVFWQELGEIFRQLQRQAAEIYNQSLIELYYEIFIKGKGFANASSVEHYLSDVCYTRAAELFKNAAIASGLRGKVKSNFRLKELKNMKSGLPTTKSDNFPIPLVKQKGGQYTGFEISSRNDDFIIKIPFGRWQVRKEIDKYRPWEKFNFEQVRKSPKPISLLLSTQRRKRNKGWSKDEGTEAEIRKVMNGDYQTSYIEVKRGSKIGEKSAWMLSLSIDVPKIDKGVDPSIIGGIDVGVKSPLVCAINNAFNRYSISDNNLFHFNKKMFARRRILLKKNRHKRAGHGAKNKLKPISILTEKSERFRKKLIERWACEIADFFIRNKVGIVQMENLESMKRKEDSYFNIRLRGFWPYAEMQNKIEFKLKQYGIEIRKVAPNNTSRTCSKCGHLNNYFSFEYRKKNKFPHFKCEKCNFKEDADYNAALNISNPKLKSTKEEL

SEQ ID NO: 2153 - protein, 726 aa, synthetic construct
SEVEFSHEYWMRHALTLAKRARDEREVPVGAILVLNNRVIGEGWNRAIGLHDPTAHAEIMALRQGGLVMQNYRLIDATLYVTFEPCVMCAGAMIHSRIGRVVFGVRNSKHGAAGSLVNVLNYPGMNHRVEITEGILADECAALLCDFYRMPRQVFNARKKAQSSINPSGSSGGSSGSVTPGTSESATPESSGGGFGGSAKNTITKTLQLRIVRPYNSAEVEKIVADEKNNREKIALEKNKDKVKEACSKHLKVAAYCTTQVERNACLFCKARKLDDKFYQKLRGQFPDAVSWQEIGEIFRQLQKQAAEIYNQSLIELYYEIFIKGKGFANASSVEHYLSDVCYTRAAELFKNAAIASGLRGKVKSNFRLKELKNMKSGLPTTKSDNFPIPLVKQKGGQYTGFEISSHNDDFIIKIPFGRWQVKKEIDKYRPWEKFDFEQVRKSPKPISLLLSTQRRKRNKGWSKDEGTEAEIRRVMNGDYQTSYIEVKRGSKIGEKSAWMLNLSIDVPKIDKGVDPSIIGGIDVGVKSPLVCAINNTFSRYSISDNDLFHYNKKMFARRRILLKKNKHKRAGHGAKNKLEPISILTEKSKRFRKKLIERWACEIADFFIKNKVGTVQIENLESMKRREDSYFNIRLRGFWPYAEMQNKIEFKLKQYGIKIRKVAPNNTSKTCSKCGHLNNYFSFEYRKKNKFPHFKCEKCNFKENADYNAALNISNPKLMSTKEEP

SEQ ID NO: 2154 - protein, 726 aa, synthetic construct
SEVEFSHEYWMRHALTLAKRARDEREVPVGAILVLNNRVIGEGWNRAIGLHDPTAHAEIMALRQGGLVMQNYRLIDATLYVTFEPCVMCAGAMIHSRIGRVVFGVRNNKHGAAGSLVNVLNYPGMSHRVEITEGILADECAALLCDFYRMPRQVFNARKKAQSSIDPGGTSGGSSGSETPGTSECATPESSGGRSGGSAKNTITKTLKLRIVRPYNSTEVEKIVADEKNNREKIALEKNKDKVKEACSKHLKVASYCTTQVERNACLFCKARKLDDKFYQKLRGQFPDAVFWQELGEIFRQLQKQAAEVYNQSLIELYYEIFIKGKGFANASSVEHYLSDVCYTRAAELFKNAAIASGLRNKIKSNFRLKELRNMKSGLPTTKSDNFPIPLVRQKGGQYTGFEISNHNGDFIIKIPFGRWQVKKEISKHRPWEKFDFEQVRKSPKPISLLLSTQRRKRNKGWSKDEGTEAEIKRVMNGDYQVSYIEVKRGSKIGEKSAWMLSLSVDVPKIDKGVDPSIIGGIDVGVKSPLVCAINNALSRYSISDNDLFHFNKKMFARRRILLRNNRHKRAGHGAKSKLKPITILTEKGERFRKKLIERWACEIANFFIKNKVGTVQMENLESMKRKEDSYFNVRLRGFWPYAEMQNKIEFKLKQYGIEIRKVAPNNTSKTCSRCGHLNNYFNFEYRRKNKFPHFKCEKCNFKENADYNAALNISNPKLKSTKEEP

SEQ ID NO: 2155 - protein, 726 aa, synthetic construct
SEVEFSHEYWMRHALTLAKRARDEREVPVGAVLVLNNRVIGEGWNRAIGLHDPTAHAEIMALHQGGLVMQNYRLIDATLYVTFEPCVMCAGAMIHSRIGRVVFGVRNSKRGAAGSLMNVLNYPGMNHCVEITEGILVDECAALLCDFYRMPRQVLNAQKKAQSSISSGGSSGGSSGSVTPGASGSVTPKSSGGSSAGSTKDTITKTLKLRIVRPYNSAEVEKIVADEKNNREKIALEKNKDKVKEACSKHLKVASYCTTQVERNACPFCKARKLDDKFYQKLRGQFPDAVFWQELGEILRQLQKQAAEIYNQSLIELYYEIFIKGRGFANASSVEHYLSDVCYTRAAELFKNAAIASGLRGKVKSNFRLKELKNMKSGLPTTKSDNFPIPLVKQKGGQYTGFEISSHNDDFIIKIPFGRWQVKKEIDKYRPWEKFDFEQVRKSPKPISLLLSTQRRKRNKGWSKDDGTEAEVRKVMNGDYRTSYIEVKRGSKTGEKSAWMLNLSIDVPKIDKGVDPSIIGGIDVGVKSPLVCAINNAFSRYSISDNDLFHFNKKMFARRRILLKKNRHKRAGHGAKNKLKPISILTEKSKRFRKKLIERWACEIADFFIKNKVGTVQMENLESMKGKEDSYFNIRLRGFWPYAEMQNKIEFKLKQYGIEIRKVAPNNTSKTCSKCGHLNNYFNFEYRKTNKFPHFKCEKCNFKEDADYNAALNISNPKLKSTKEEP

SEQ ID NO: 2156 - protein, 726 aa, synthetic construct
SEVEFSHEYWMRHALTLARRARDEREVPVGAILVLNNRVIGEGWNRAIGLHDPTAHAEIMALRQGGLVMQNYRLTDATLYVTFEPCVMCAGAMVHSRIGRVVFGVRNSKRGAAGSLMNVLNYPGMSHCVEITEGILVDECAALLCDFYRMPRQVLNAQKKAQSSISSGGSSGDSGGGETPGASESVTPKSSGGSSAGSTKNTITKTLKLRIVRPYNSAEVEKIVADEKNNREKIALEKNKDKVQEACSKHLKVASYCTTQVERNACLFCKARKLDDKFYQKLRGQFPDAVFWQEIGEIFRQLQKQAAEIYNQSLIELYYEIFIKGKGFANASSVEHYLSDVCYTRAAELFKNAAIASGLRGKVKSNFRLKELKNMKSGLPTTKSDNFPIPLVRQKGGRYTGFEISSHNDDFIIKVPFGRWQVKKEIDKYRPWEKFDFEQVRKSPKPISLLLSTQRRKRNKGWSKDEGTEAEIRKVMNGDYQTSYIEVKRGSKIGEKSAWMLNLSIDVPKIDKGVDPSIIGGIDVGVKSPLVCAINNTIGRYSISDNDLFRFNKKMFARRRILLKKNRHKRAGHGAKNKLKPISILTEKSGRFRKKLIERWACEIADFFIKNKVGTVQMENLEGMKRREDSYFNIRLRGFWPYAEMQNKIEFKLKQYGIEVRKVAPNNTSKTCSKCGHLNNYFNFEYRKKNKFPHFKCVKCNFKEDADYNAALNISNPKLKSTKEEP

SEQ ID NO: 2157 - protein, 726 aa, synthetic construct; identical to SEQ ID NO: 684

SEQ ID NO: 2158 - protein, 726 aa, synthetic construct; identical to SEQ ID NO: 684

SEQ ID NO: 2159 - protein, 726 aa, synthetic construct
SEVEFSHEYWMRRALTLAKRARDEREVPVGAVLVLNNRVIGVGWNRAVGLHDPTAHAEIMALRQGGLVMQNYRLIEATLYVTFEPCIMCAGAMIHSRIGRVVFGVRNSKRGAAGSLMNVLNYPGMNHRVEITEGILADECAALLCDFYCMPRQVLNAQKKARSCINSGGSSGGSSGSETPGAGESVTPKSSVGSSAGSTKNTITKTLKLRIVRPYNSAEVEKIVADEKNNREKIALEKNKDKVKEACSKHLKVAAYCTTQVERNACLFCKARKLDDKFYQKLRGQFPDAVFWQEIGEIFRQLQKQAAEIYNRSLIELYYEIFIKGKGFANASSVEHYLSDVCYTRAAELFKNAAIASGLRGKVKSNFRLKELKNMKSGLPTTKSDNFPIPLVKQKGGQYTGFEINSHNDDFIIKIPFGRWQVKKEINKYRPWEKFDFEQVRKSPKPISLLLSTQRRKRNKGWSKDEGTEAEIRKVMNGDYQTSYIEVKRGSKIGEKSAWMLNLSIDVPKIDKGVDPSIIGGIDVGVKSPLVCAINNALSRYSISDNDLFHFNKKMFARRRILLKKNRHKRAGHGARNKLKPVAVLTEKSKRFRKKLIERWACEIANFFIKNKVGTVQMENLESMKRKEDSYFNIRLRGFWPYAEMQNKIEFKLRQYGIEIRKVAPSNTSKTCSKCGHLNNYFNFEYRKKNKFPYFKCEKCNFKENADYNAALNISNPKLKSTKEEP

SEQ ID NO: 2160 - protein, 726 aa, synthetic construct; identical to SEQ ID NO: 684

SEQ ID NO: 2161 - protein, 726 aa, synthetic construct
SEVEFSHEYWMRHALTLAKRARDEREVPVGAVLVLNNRVIGEGWNRAIGLHDPTAHAEIMALRQGGLVMQNYRLVDATLYVTFEPCVLCAGAMVHSRIGRVVFGVRNSKRGAAGSLMNVLNYPGMNHRVEITEGILADECAALLCDFYRMPRQVFNARKKARSNINSSGPSGGSSCSETPGASESPTPESSGGIPSGSAKNTITKTLKLRVVRPYNSAEVEKIVADEKNNREKIALEKNKDKVKEACSKHLKVAAYCTTQVERNACLFCKARKLDDKFYQKLRGQFPDAVFWQEIGEIFRQLQKQAAEIYNQSLIELYYEIFIKGKGFANASSVEHYLSDVCYTRAAELFKNAAIASGLRGKVKSNFRLKELKNMKSGLPTTKSDNFPIPLVKQKGGQYTGFEISSHNDDFVIKIPFGRWQVKEEIDKYRPWEKFDFEQVRKNPKPISLLLSTQKRKRNKGWSKDEGTEAEIRKVMNGDYQTSYIEVKRGSKIGEKSAWMLNLSIDVPKIDKGVDPSIIGGIDVGVKSPLVCAINNALSRYSISDNDLFHFNKKMFARRRILLRKNRHKRTGHGAKNKLKPITIMTEKSKRFRKKLIERWACEIADFFIKNKVGTVQMENLESMKRKEDSYFNIRLRGFWPYAEMQNKIEFKLKQYGIEIRKVAPYNTSKTCSRCGHLNNYFNFEYRRKNKFPHFKCEKCNFKENADYNAALNISNPKLKSTKEEP

SEQ ID NO: 2162 - protein, 726 aa, synthetic construct
GEVEFSHEYWMRRALTLAKRARDEREVPVGAVLVLNNRVIGVGWNRAVGLHDPTAHAEIMALRQGGLVMQNYRLVEATLYVTFEPCVMCAGAMIHSRIGRVVFGVRNNKHGAAGSLVNVLNYPGMNHRVEITEGILADECTALLCDFYRMPRQVFNARKKAQSSISPDGSSDGSSGSETPGTSESATPESSGGGSSGSAKNTITKTLQLRIVRPYNSAEVEKIVADEKNNREKIALEKNKDKVREACNKHLKVASYCTTQVERNACPFCKARKLDDKFYQKLRGQFPDAVFWQELGEILRQLQKQAAEIYNQSLIELYYEIFIKGKGIANASRVEHYLSDVCYTRAAELFKNAAIASGLRSKIKSNFRLKELRNMKSGLPTTMSDNFPIPLVKQKGGQYTGFEISSHNSDFVVKIPFGRWRVKEEIDKYRPWEKFDFEQVRKSPKPIRLLLSTQRRKKNKGWSKDEGTEAEIRRVMNGDYQTSYIEVKRGSKIGEKSAWMLNLSIDVPKIDKGVDPSIIGGIDVGVKSPLVCAINNSFSRYSISDNDLFRFNKKMFARRRILLKKSKHKRAGHGAKNKLKPISILTEKSKRFRKKLIERWACEIADFFIKNKVGTVQMENLESMKRKEDSYFNIRLRGFWPYSEMQNKIEFKLKQYGIEIRKVAPNNTSKTCSKCGHLNNYFNFEYRKKNKFPHFKCEKCNFKEDADYNAALNISNPKLKSTKEEP

SEQ ID NO: 2163 - protein, 726 aa, synthetic construct
SEVEFSHEYWMRHALTLAKRARDEREVPVGAVLVLNNRVIGEGWNRAIGLHDPTAHAEIMALRQGGLVMQNYRLTDATLYVTFEPCVMCAGAMIHSRIGRVVFGVRNSKRGAAGSLMNVLNYPGMNHCVEITEGILVDECAALLCDFYRMPRQVLNAQKKAQSSINPSGSSGGSSGSVTPGTSESATPESSGGGSSGSAKNTITKTLQLRIVRPYNSAEVEKIVADEKNNREKIALEKNKDKVKEACSKHLKVAAYCTTQVERNACPFCKARKLDDKFYQKLRGQFPDAVFWQELGEILRQLQKQAAEIYNQSLIELYYEIFIKGRGFANASSVEHYLSDVCYTRAAELFKNAAIASGLRGKVKSNFRLKELKNMKSGLPTTKSDNFPIPLVKQKGGQYTGFEISSHNSDFIIKIPFGRWQEKEEIDKYRPWEKFDFAQVRKSPKPISLLLSTQRRKRNKGWSNDEGTEAEIRKVMNGDYQTSYIEVKRGSKIGEKSAWMLSLSIDVPKIDKGVDPSIVGGIDVGVKSPLVCAINNALGRFSISDNDLFHFNKKMFARRRILLRKNRHKRAGHGAKNKLKPISILTEKSRRFRKKLIERWACEIADFFIKNKVGTVQMEDLESMKRRGDSYFNIRLRGLWPYAEMQNKIEFKLKQYGIEIRKVAPNNTSKTCSKCGHLNNYFNFEYRKKNKFPHFKCEKCNFKENADYNAALNISNPKLKNTKEEP

SEQ ID NO: 2164 - protein, 726 aa, synthetic construct
SEVEFSHEYWMRHALTLAKRARDEREVPVGAILVLNNRVIGEGWNRAIGLHDPTAHAEIMALRQGGLVMQNYRLVDATLYVTFEPCVMCAGAMIHSRIGRVVFGVRNNKHGAAGSLVNVLNYPGMNHRVEITEGILADECAALLCDYYRMPRQVFNARKKAQSSINSGSSSDGGSGSETPGTSESATPESSGGSSGGSAKNTITKTLKLRIVRPYNSAEVEKIVADEKNNREKIALEKNKDKVKEACSKHLKVAAYCTTQVERNACLFCKARRLDDKFYQKLRGQFPDAVFWQEIGEIFRQLQKQAAEIYNQSLVELYYEVLIKGKGIANASSVEHYLSDVCYTRAAGLFKNAAIASGLRNKIKSNFRLKELRNMKSGLPTTKSDNFPIPLVRQKGGRYTGFEISNHNGDFIIKIPFGRWQAKKEINKHRPWEKFDFEQVRKSPKPISLLLSTQRRKRNKGWSKDEGTEAEIRKVMNGDYQTSYIEVKRGSKIGEKSAWMLNLSIDVPKIDKGVDPSIIGGIDVGVKSPLVCAINSALSRYSISDNDLFHFNKKMFARRRILLRKNRHKRAGHGARNKLKPITVLTEKSERFRKKLIERWACEIANFFIKNKVGTVQMENLESMKRREDSYFNIRLRGFWPYAEMQSKIEFKLKQYGIEVRKVAPNNTSKSCSKCGHLNNYFNFEFRKKNKFPHFKCEKCNFKEDADYNAALNISNPKLKSTKEEP

SEQ ID NO: 2165 - protein, 726 aa, synthetic construct
SEVEFSHEYWMRHALTLAKRARDEREVPVGAVLVLNNHVIGEGWNRAIGLHDPTAHAEIMALRQGGLVMQNYRLSDATLYVTFEPCVMCAGAMIHSRIGRVVFGVRNSKRGAAGSLMNVLNYPGMNHCVEITEGILVDECAALLCDFYRMPRQVLSAQKKAQSSVSSGDSSGGSSGSETPGASGSVTPKSSVGSSAGSTKSTITKTLKLRIVRPYNSAEVEKIVADEKNNREKIALEKNRDKVKEACSKHLKVAAYCTTQVERNACLFCKARKLDDKFYQKLRGQFPDAVFWQEIGEIFRQLQKQAAEIYNQSLIELYYEIFIKGKGFANASSVEHYLSDVCYTRAAELFKNAAIASGLRGKVKSNFRLKELKNMKSGLPTTKSDNFPIPLVKQKGGQYTGFEISSHNDDFIIKIPFGRRQVKKEIDKYRPWEKFDFEQVRKSPKPISLLLSTQRRKRNKGWSKDEGTEAEIRKVMNGDYQTSYIEVKRGSKIGEKSAWMLNLSIDVPKIDKGVDPSIIGGIDVGVKSPLVCAINNAFSRYSIGDNDLFRFNKKMFARRRVLLKKNRHKRAGHGAKNKLKPISILTGKSERFRKKLIERWACEIADFFIKNKVGTVQMENLESMKRKEDSYFNIRLRGFWPYAEMQNKIEFKLKQYGIEIRKVAPNNTSKTCSKCGHLNNYFNFEYRRKNKFPHFKCEKCHFKEDADYNAALNISNPKLRCTKEEP

SEQ ID NO: 2166 - protein, 726 aa, synthetic construct
SEVEFSHEYWMRHALSLAKRARDEREVPVGAVLVLNNRIIGEGWNRAIGLHDPTAHAEIMALRQGGLVMQNYRLTDATLYVTFEPCVMCAGAMIHSRIGRVVFGVRNSKRGAAGSLMNVLNHPGMNHCVEITEGILVDECAALLCDFYRMPRQVLNAQKKAQSSISPGGSSGGSSGSETPGASESVTLKNSGGSSGGSAKNTITKTLQLRIVRPYNSAEVEKIVADEKNNREKIALEKNRDKVKEACSKHLKVAAYCTTQVERNACLFCKARRLDDKFYQKLRGQFPDAVFWQEIGEIFRQLQRQAAEIYNQSLIELYYEIFIKGKGFANASSVEHYLSDVCYTRAAELFKNAAIASGLRGKVKSNFRLKELKNMKSGLPTTKSDNFPIPLVKQKGGQYTGFEISSRNDDFIIKIPFGRWQVKKEIDKYRPWEKFDFEQVRKSPKPISLLLSTQRRKRNKGWSKDEGTEAEIRKVMNGDYQTSYIEVKRGSKIGEKSAWMLNLSIDVPKIDKGVDPSIIGGIDVGVKSPLVCAINNAFSRYSISDNDLFHFNKKMFARRRILLKKNRHKRAGHGAKNKLKPIFILTEKSKRFRKKLIEKWACEIADFFIKNKVGTVQMENLESMKRKEDSYFNIRLRGFWPYAEMQNKIEFKLKQYGIEIRKVAPNNTSKTCSKCGHLNNYFDFEYRKKNKFPHFKCEKCNFKENADYNAALNISNPELKSTKEEP

SEQ ID NO: 2167 - protein, 726 aa, synthetic construct; identical to SEQ ID NO: 684

SEQ ID NO: 2168 - protein, 726 aa, synthetic construct
SEIEFSHEYWMRHALTLARRARDEREVPVGAILVLNNRVIGEGWNRAIGLHDPTAHAEIMALRQGGLVMQNYRLIDATLYVTFEPCVMCAGAMIHSRIGRVVFGVRNNKHGAAGSLVNVLDYPGMNHRVEITEGILADECAALMCDFYRMPRQVFNARKKAQSSISPGGSSGGSSGSETPGTSESATPESSDGSSGGSAKNTITKTLKLRIVRPYNCAEVEKIVADEKNNREKIALEKNKDKVKEACSKHLKVAAYCTTQVERNACLFCKARKLDDKFYQKLRGQFPDAVFWQEIGEVFRQLQKQAAEIYNQSLIELYYEIFIKGKGFANASSVEHYLSDVCYTRAAELFKNAAIASGLRGKVKSNFRLKELKNMKSGLPTTKSDNFPIPLVKQKGGQYAGFEISSHNDDFIIKIPFGRWQVKKEIDKYRPWEKFDFEQVRKSPKPISLLLSTQRRKRNKGWSKDEGTEAEIRKVMNGDYQTSYIEVKRGSKIGEKSAWMLSLSIDVPKIDKGVDPSTIGGIDVGVKSPLVCAINNAFCRYSISDNDLFHFNKKMFARRRILLKKSRHKRAGHGAKNKLKPISILTEKSKRFRKKLIERWACEIADFFIKNKVGTVQMENLESMKRKEDSYFNIRLRGFWPYAEMQNKIEFKLKQYGIEIRKVAPNNTSKTCSKCGHLNNYFNFEYRKKNKFPHFKCEKCNFKENADYNAALNISNPKLKSTKEEP

SEQ ID NO: 2169 - protein, 726 aa, synthetic construct
SGVEFSHEYWMRHALTLAKRARDEREVPVGAVLVLNNRVIGEGWNRAIGLHDPAAHAEIMALRQGGLVMQNYRLIGATLYVTFEPCVMCAGAMIHSRVGRVVFGVRNNKHGAAGSLVNVLNYPGMNHRVEITEGILADECAALLCDFYRMPRQVFNARKKAQSGINPGGSSGGSSGSETPGTSESATPESSGGSSGGSAKNTITKTLKLRIVRPYNSAEVEKIVADEKNNRERIALEKNKGKVKEACSKHLKVAAYCTTQVERNACLFCKARKLDDKFYQKLRGQFPDAVFWQEIGEIFRQLQRQAAEVYNQSLIELYYEIFIKGKGIANASSVGHYLSDVCYTRAAELFKNAAIASGLRGKVKSNFRLKELKNMKSSLPTTKSDNFPIPLVKQKGGQYTGFEISSHNDDFIIKIPFGRWQVKKEIDKYRPWEKFNFEQVRKSPKPISLLLSTQRRKRNKGWSKDEGTEAEIRKVMNGDYQTSYIEVKRGSKIGEKSAWMLNLSIDVPKIDKGVNPSIIGGIDVGVKSPLVCAINNSSSRYSICDNDLFRFNKKMFARRRILLKKNRHKRAGHGAKNKLKPITVLTEKSERFRKKLIERWAREIANFFIKNKVGTVQMENLESMKRREDSYFNIRLRGFWPYAEMQNKIEFKLKQYGIEIRKVAPNNTSKTCSKCGHLNNYFNFEFRKKNKFPHFKCEKCNFKENADYNAALNISNPKLKSTKEEP

SEQ ID NO: 2170 - protein, 726 aa, synthetic construct
SEVEFSHEYWMRHALMLAKRARDEREVPVGAVLVLNNRVIGEGWNRAIGLHDPTAHAEIMALRQGGLVMRNYRLTDATLYVTFEPCIMCAGAMIHSRIGRVVFGVRNSKRGAAGSLMNVLNYPGMNHCVEITEGILVDECAALLCDFYRMPRQVLNAQKKAQSSINPGGSSGGSSGSETPGTSESVTPESSGGSSGSSAKNTITKTLKLRIVRPYNSAEVEKIVADEKNNREKIALEKNKDKVKEACSKHLKVASYCTTQVERNACPFCKARKLDDKFYQKLRGQFPDAVFWQELGEILRQLQKQAAEIYNQSLIELYYEIFIKGKGIANASNVEHYLSDVCYTRAAELFKNAAIASGLRNKIKSNFRLKELRNMKSGLPTTKSDNFPIPLVRQKGGQYTGFGISNHNGDFIIKIPFGRWQVKKEIDKYRPWERFDFEQVRKSPKPISLLLSTQRRKRNRGWSKDEGTEAEIRKVMNGDYQTSYIEVKRGCKIGEKSAWMLNLSIDVPKIDKGVDPSIIGGIDVGVKSPLVCAINNAFSRYSISDNDLFRFNKKMFARRRILLEKNRHKRAGHGVKNKLKPITILTEKSGRFRKKLIERWACEIADFFVKNKVGTVQMENLESMKRKEDSYFNIRLRGFWPYAEMQNKIEFKLKQYGIEIRKVAPNNTSKTCSKCGHLNNYFNFEYRKKNKFPHFKCEKCNFKENADYNAALNISNPKLKSTREEP

SEQ ID NO: 2171 - protein, 726 aa, synthetic construct
SEVEFSHEYWMRHALTLAKRARDEREVPVGAILVLNNRVIGEGWNRAIGLHDPTAHAEIMALRQGGLVMQNYRLIDATLYVTFEPCVMCAGAMIHSRIGRVVFGVRNSKRGAAGSLMNVLNYPGMNHCVEITEGILVDECAALLCDFYRMPRQVLNAQKKAQSSISPGGSSGGSSGSGTPGASESVAPKSSVGSSAGSTKNTTTKTLKLRIVRPYNSAEVEKIVADEKNNREKTALEKNKDKVKEACSEHLKVAAYCTTQVERSACLFCKARKLDDKFYQKLRGQFPDAVFWQELGEILRQLQKQAAEIYNQSLVELYYEILIKGKGIANASSVEHYLSDVCYTRAAKLFKNAAIASGLRGKIKSNFRLKELRNMKSGLPTTKSDNFPIPLVKQKGGQYTGFEISSHNGDFIIRIPFGRWQVKKEIDKYRPWEKFDFEQVRKSPKPISLLLSTQRRKRNKGWSKDEGTEAEIRKVMNGDYQTSYIEVKRGSKIGEKSAWMLNLSIDVPKIDKGVDPSIIGGIDVGVKSPLVCAINNAFSRYSISDNDLFHFNKKMFARRRILLKKNRHKRAGHGAKNKLKPITILTEKSVRFRKKLIERWACEIADFFIKNKVGTVQMENLESMKRKEDSYFNIRLRGFWPYAEMQNKIEFKLKQYGIETRKVAPNNTSKTCSKCGHLNNYFNFEYRKKNKFPHFKCEKCNFKENADYNAALNISNPKLKSTKGEP

SEQ ID NO: 2172 - protein, 726 aa, synthetic construct
SEVEFSHEYWMRHALTLAKRARDEREVPVGAILVLNNRVIGEGWNRAIGLHDPTAHAEIMALRQGGLVMQNYRLIDATLYVTFEPCVMCAGAMIHSRIGRVVFGVRNNKHGAAGSLVNVLNYPGMNHRVEITEGILADECAALLCDFYRMPRRVFNARKKAQSSINPGGPSGGSSGSETPGTSESATPESSGGSSGGSAKNTITKTLKLRIVRPYNSAEVEKIVADEKNSREKIALERNKDKVKEACSEHLKVAAYCTTQVERNACLFCKARKLDDRFYQKLRGQFPDAVFWQETGEIFRQLQRQAAEIYNQSLIELYYEIFIKGKGFANASSVEHYLSDVCYTRAAELFKNAAIASGLRGKVKSNFRLKELKNMKSGLPTTKSDNFPIPLVKQKGGQYTGFEISSHNDDFIIKIPFGRWQVKGEIDKYRPWEKFDFEQVRKSPKPISLLLSTQRRKRNKGWSKDEGTEAEIRKVMNGDYQTSYIEVKRGSKIGEKSAWMLNLSIDAPKIDKGVDPSIIGGIDVGVKSPLVCAINNALSRYSISDNDLFHFNKKMFARRRILLRKNRHKRAGHGAKNKLKPITIMTEKSKRFRKKLIERWACEIADFFIKNKVGTVQMENLESMKRREDSYFNIRLRGFWPYAEMQNKIEFKLKQYGIVVRKVAPNNTSKTCSKCGHLNNYFNFEYRKKNKFPHFKCEKCNFKEDADYNAALNISNPKLKSTKGEP

SEQ ID NO: 2173 - protein, 726 aa, synthetic construct
SEVEFSHEYWMRHALTLAKRARDEREVPVGAILVLNNRVIGVGWNRAIGLHDPTAHAEIMALRQGGLVMQNYRLIDATLYVTFEPCVMCAGAMIHSRIGRVVFGVRNSKHGAAGSLVNVLNCPGMNHRVEITEGILADECAALLCDFYRMPRQVFNARKKAQSSINSGGSSGGSSGSETPGTSESATPKSSGGSSGGSAKNTITKALKLRIVRPYNSAEVEKIVADEKNNRERIALEKNKDKVKEACGKHLKVAAYCTTQVERNACLFCKARKLDDKFYQKLRGQFPDAVFWQEIGEIFRQLQKQAAEIYNQSLIELYYEILIKGKGFANASSVEHYLSDVCYTRAAELFKNAAIASGLRGKVKSNFKLKELRSMRSGLPTTKSDNFPIPLVKQKGGQYTGFEISSHNDDFIIKIPFGRWQVKKEIDKYRPWEKFDFEQVRKSPKPISLLLSTQRRKRNKGWSKDEGTEAEIKKVMNGDYQTSYIEVKRGSKTGEKSAWMLNLSIDVPKIDKGVDPCIIGGIDVGVKSPLVCAINNAFSRYSISDNDLFHFNKKMFARRRILLKKNRHRRAGHGARNKLKPITVLTEKSKRFRKKLIERWACEIANFFIKNKVGTVQMENLESMKRKEDSYFNIRLRGLWPYAEMQNKIEFKLKQYGIEIRKVAPNNTSKTCSKCGHLNNYFNFEYRKRNKFPHFKCEKCNFKENADYNAALNISNPKLKGTKEEP

SEQ ID NO: 2174 - protein, 726 aa, synthetic construct
SEVEFSHEYWMRHALTLAKRARDEREVPVGAILVLNNRVIGEGWNRAIGLHDPTAHAEIMALRQGGLVMQNYRLIDATLYVTFEPCVMCAGAMIHSRIGRVVFGVRNSKHGAAGSLVNVLNYPGMNHRVEITEGILADECAALLCDFYRMPRQVFNARKKAQSSINPSGSSGGSSGSVTPGTSESATPESSGGGFGGSAKNTITKTLQLRIVRPYNSAEVEKIVADEKNNREKIALEKNKDKVKEACSKHLKVAAYCTTQVERNACLFCKARKLDDKFYQKLRGQFPDAVSWQEIGEIFRQLQKQAAEIYNQSLIELYYEIFIKGKGFANASSVEHYLSDVCYTRAAELFKNAAIASGLRGKVKSNFRLKELKNMKSGLPTTKSDNFPIPLVKQKGGQYTGFEISSHNDDFIIKIPFGRWQVKKEIDKYRPWEKFDFEQVRKSPKPISLLLSTQRRKRNKGWSKDEGTEAEIKKVMNGDYQTSYIEVKRGSKIGEKSAWMLNLSIDVPKIDKGVDPRIIGGIDVGVKSPLVCAINNVLSRYSISDNDLFHFNKKMFARRRILLKKNGHKRAGHGAKNKLKPITIMTEKSKRFRKKLIERWACEIADFFIKNKVGTVQMENLESMKRKEDSYFNIRLRGFWPYAEMQNKIEFKLKQYGIVVRKVAPNNTSKTCSQCGHLNNYFNFEYRKKNKFPHFKCEKCNFKEDADYNAALNISNPKLKSTKEEP

SEQ ID NO: 2175 - protein, 726 aa, synthetic construct
SEVEFSHEYWMRHALTLAKRARDEREVPVGAVLVLNNRVIGGGWNRAIGLHDPTAHAEIMALRQGGLVMQNCRLADATLYVTFEPCVMCAGAMIHSRIGRVVFGVRNSKRGAAGSLMNVLNYPGMNHRVEITEGILADECAALLCDFYCMPRQVFNARKKAQSSINPGGSSGGSGGSETPGTSESPTPESSGGSSGGSAKNTITKTLKLRIVRPYNSAEVEKIVADEKNNREKIALEKNKDKVKEACSKHLKVAAYCTTQVERNACLFCKARKLDDKFYQKLRGRFPDAVFWQEISEIFRQLQKQAAEIYNQSLIELYYEIFIKGKGFANASGVEHYLSDVCYTRAAELFKNAAIASGLRGKVKSNFRLKELKNMKSGLPTTKSDNFPIPLVKQKGGQYTGFEISSHNDDFIIKIPFGRWRGKKEVDKYRPWEKFDFEQVRKSPKPISLLLSTQRRKRNKGWSKDEGTEAEIKKVMNGDYQTSYIEVKRGSKIGEKSAWMLSLSIDVPKIDRGVDPSIIGGIDVGVKSPLVCAINNASSRLSISDNDLFRFNKKMFARRRILLKKNGHKRAGHGAKNKLKPITILTEKSVRFRKKLIERWACEIADFFIRNKVGTVQMENLESMKRREDSYFNIRLRGFWPYAEMQNKIEFKLKQYGIEIRKVAPNNTSKTCSKCGHLNNYFNFEYRKKNKFPHFKCEKCNFKENADYNAALNISNPKLRSTKEEP

SEQ ID NO: 2176 - protein, 726 aa, synthetic construct
SEVEFSHEYWMRHALTLAKRARDEREVPVGAILVLNNRVIGEGWNRAIGLHDPTAHAEIMALRQGGLVMQNYRLIDATLYVTFEPCVMCAGAMIHSRIGRVVFGVRNNKHGAAGSLVNVLNYPGMNHRVEITEGILADECAALLCDFYRMPRQVLNAQKKAQSSISSGGSSGGSSGSETPGASGSVTPKSSGGSSAGSTKDTITKTLKLRIVRPYNSAEVEKVVADEKNNREKIAMEKNKDKVKEACSKHLKVASYCTTQVERNACLFCKARKLDDKFYQKLRGQFPDAVFWQELGEIFRQLQKQAAEIYNQSLIELYYEIFIKGKGFANASSVEHYLSDVCYSRAAELFKNAAIASGLRGKVKSNFRLKELKNMKSGLPTTKSDNFPIPLVKQKGGQYTGFEISSHNDDFIIKIPFGRWQVKKEIDKYRPWEKFDFEQVRKSPKPISLLLSTQRRKRNKGWSKDEGTEAEIRKVMNGDYQTSYIEVKRGSKIGEKSAWMLNLSIDVPKIDKGVDPSIIGGIDVGVKSPLVCAINNAFGRYSISDNDLFHFNKKMFARRRILLKKNRHKRAGHGAKNKLKPITILTEKSKRFRKKLIERWACEIADFFIKNKVGTVQMENLGSMKRKEDSYFNIRLRGFWPYAEMQNKIEFKLKQYGIEIRKVAPDNTSKTCSKCGHLNNYFNFEYRKKNKFPHFKCEKCNFKEDADYNAALNISNPKLKSTKEEP

SEQ ID NO: 2177 - protein, 726 aa, synthetic construct
SEVEFSHEYWMRRALTLAKRARDEREVPVGAVLVLNNRVIGVGWNRAVGLHDPTAHAEIMALRQGGLVMQNYRLTDATLYVTFEPCVMCAGAMIHSRIGRVVFGVRNSKRGAAGSLMNVLNYPGMNHCVEITEGILVDECAALLCDFYRMPRQVLNAQKKAQPSISSGGSSGGSSGSETSGASESVTPKSSGGGSAGSTKNTITKTLKLRIVRPYNSAEVEKIVADEKNSREKIALEKNKDKVKEACSRHLKVAAYCTTQVERNACPFCKARKLDDKFYQELRGQFPDAVFWQELGEILRQLQKQAAEVYNQSLIELYYEIFIKGKGFANASSVEHYLSDVCYTRAAELFKNAAIASGLRGKVKSNFRLKELKNMKSGLPTTKSDNFPIPLVKQKGGQYTGFEISSHNDDLIIKIPFGRWWVKKEIDKYRPWEKFDFEQVRKSPKPISLLLSTQRRKRNKGWSKDEGTEAEIKKVMNGDYQTSYIEVKRGSKIGEKSAWMLNLSIDVPKIDKGVDPSIIGGIDVGVKSPLVCAINNAFSRYSIGDNDLFRFNKKMFARRRILLEKNRHKRAGHGVKNKLKPITILTEKSRRFRKKLIERWACEIADFFVKNKVGTVQMENLEGMKRKEDSYFNIRLRGFWPYAEMQNKIEFKLKQYGIKVRMVAPNNTSKTCSKCGHLNNYFSFEYRKKNKFPHFKCKKCNFKENADYNAALNISNPKLKSTKEEP

SEQ ID NO: 2178 - protein, 726 aa, synthetic construct
SEVEFSHEYWMRHALTLAKRARDEREVPVGAILVLNNRVIGEGWNRAIGLHDPTAHAEIMALRQGGLVMQNYRLTDATLYATFEPCVMCAGAMIHSRIGRVVFGVRNSKHGAAGSLMNVLNYPGMNHRVEITEGILADECAGLLCDFYRMPRQVFSARKKAQSSINPGGSSGGSSGGKAPGTSESATLESSGGSSGGSAKNSITKTLKLRIVRPYNSAEVEKIVADEKNNREKTALEKNKGKVKEACSKHLKVATYCTTQVERNACLFCKARKLDDKFYQKLRGQFPDAVFWQEIGEIFRQLQKQAAEIYNQSLIELYYEIFIEGKGSASASRVEHYLSDVCYTRAAELFKNAAIASGLRNKIKSNFRLKELRNMRSGLPTTKSDNFPIPLVKQKGGQYTGFEISSHNDDFIIKIPFGRWQVKKEIDKYRPWEKFDFEQVRKSPKPISLLLSTQRRKRNKGWSKDEGTEAEIRKVMNGDYQTSYIEVKRGSKIGEKSAWMLNLSIDVPKIDKGVDPSIIGGIDVGVKSPLVCAINNAFCRYSISDNDLFHFNKKMFARRRILLKRSRHKRAGHGAKNKLKPISILTEKSKRFRKKLIERWACEIADFFIKNKVGTVQMENLESMKRKEDSYFNIRLRGFWPYAEMQNKIEFKLKQYGIEIRKVAPNNTSKTCSKCGHLNNYFNFEYRKMNKFPHFKCEKCNFKENADYNAALNISNPKLKSTKEEP

SEQ ID NO: 2179 - protein, 726 aa, synthetic construct
SEVEFSHEYWMRHALTLAKRARDEREVPVGAVLVLNNRVIGEGWNRAIGLHDPTAHAEIMALRQGGLVLQNYRLVDATLYVTFEPCVLCAGAMVHSRIGRVVFGARNSKRGAAGSLMNILNYPGMNHRVEITEGILADECAALLCDFYRMPRQVFNAQKKAQSSINSGGSSGGSSGSETPSTSESATPESSGGSSGGSAKNTITKTLQLRIVRPYNSAEVEKIVTDEKNNREKIALEKNKDKVKEACSKHLKMASYCTTQVERNACLFCKARKLDDKFYQKLRGQFPDAVFWQELGGIFRQLQKQAAEIYNQSLIELYYEIFIKGKGITNASRVEHYLSDVCYTRAAELFKNAAIASGLRSKVRSNFRLKELKNMRSGLPTTKSDNFPIPLVKQKGGQYTGFEISSHNDDFIIKIPFGRWQVKKEIDKYRPWEKFDFEQVRRSPKPISLLLSTQRRKKNKGWSKDEGTEAEIRRVMNGDYQTSYIEVKRGSKIGEKSAWMLNLSIDVPRIDKGVDPSIIGGIDVGVKSPLVCAINNAFSRYSISDNDLFHFNKKMFARRRILLRKNRHKRAGHGAKNKLKPISILTGKSERFRKKLIERWACEIADFFIKNKVGTVQMENLEGMKRKEDSYFNIRLRGFWPYAEMQNKIEFKLKQYGIEIRKVAPNNTSKTCSECGHLNNYFNFEYRKKNKFPHFKCEKCNFKENADYNAALNISNPKLKSTKEEP

SEQ ID NO: 2180 - protein, 726 aa, synthetic construct
SEVEFSHEYWMRHALTLAKRARDEREVPVGAVLVLNNRVIGEGWNRAIGLHDPTAHAEIMALRQGGLVMQNYRLTDATLYVTFEPCVMCAGAMVHSRIGRVVFGVRNSKHGAAGSLVNVLNYPGMNHRVEITEGILADECAALLCDFYRMPRQVFNARKKAQSSINSGGSSDGGSGSETPGTSESATPESSGGSSGGSAKNTITKTLKLRIVRPYNSAEVEKIVADEKNNREKIALEKNKDKVKEACSEHLKVAAYCTTQVERSACLFCKARKLDDKFYQELRGQFPDAVFWQEIGEIFRQLQKQAAEIYNQSLIELYYEIFIKGKGFANASSVEHYLSDVCYTRAAELFKNAAIASGLRGKVKSNFRLKELKNMKSGLPTTKGDNFPIPLVKQKGGQYTGFEISSHNDDFIVKIPFGRWQVKKEIDKYRPWEKFDFEQVRKSPKPISLLLSTQRRKRNKGWSKDEGTEAEIKKVMNGDYQTSYIEVKRGRKTGEKSAWMLNLSIDVPKIDKGVDPSIIGGIDVGVKSPLVCAINNALSRYSISDNDLFHFNKKMFARRRILLRKNRHKRAGHGARNKLKPISILTEKSKRFRKKLIERWACEIADFFIKNKVGTVQMENLESMKRKEDSYFNIRLRGFWPYAEMQNKIEFKLKQYGIEIRKVAPNNTSKTCSKCGHLNNYFNFEYRKKNKFPHFKCEKCSFKENADYNAALNISNPKLKSTKEEP

SEQ ID NO: 2181 - protein, 726 aa, synthetic construct
SEVEFSHEYWMRHALTLAKRARDEREVPVGAVLVLNNRVIGEGWNRAIGLHDPTAHAEIMALRQGGLVMQNYRLVDATLYVTFEPCVLCAGAMVHSRIGRVVFGVRNNKRGAAGSLMNILNYPGMSHRVEITEGILADECAALLCDFYRMPRQVFNAQKKARSNINSGGSSGGSSGSETPGTSESPTPESSVGSPAGSTKNTITKTLKLRIVRPYNSAEVEKIVADEKNNREKIALEKNKDKVKEACSKHLKVAAYCTTQVERNACLFCKARKLDDKFYQKLRGQFPDAVFWQEISEIFRQLQKQAAEIYNQSLIELYYEIFIKGKGFANASSVEHYLSDVCYTRAAELFKNAAIASGLRGKVKSNFRLKELKNMKSGLPTTKSDNFPIPLVKQKGGQYTGFEISSHNDDFIIKIPFGRWQVKKEIDKYRPWEKFDFEQVRKSPKPISLLLSTQRRKRNKGWSKDEGTEAEVRKVMNGDYQTSYIEVKRGSKIGEKSAWMLNLSIDVPKIDKGVDPSIIGGIDVGVKSPLVCAINNAHSRYSISDNDLFHFNKKMFARRRILLKKNRHRRAGHGARNKLKPITVLTEKSRRFRKKLIERWACEIANFFIKNKVGTVQMENLESMKRKEDSYFNIRLRGFWPYAEMQNKIEFKLKQYGIEIRKVAPNNTSKTCSKCGHLNNYFSFEYRKKNKFPHFKCEKCNFKEDADYNAALNISNPKLKSTKEEP

SEQ ID NO: 2182 - protein, 726 aa, synthetic construct
SEVEFSHEYWMRHALTLAKRARDEREVPVGAVLVLNNRVIGEGWNRAIGLHDPTAHAEIMALRQGGLVMQNYRLIDATLYVTFEPCVMCAGAMIHSRIGRVVFGVRNSKHGAAGSLVNVLNYPGMNHRVEITEGILADECAALLCDFYRMPRQVFGARRKAQSSINPGGSSGGSSGSETPGASESVTPKSSGGSSGGSAKNTITKTLKLRIVRPYNSAEVEKIVADEKNNREKIALEKNKDKVKEACSKHLKVAAYCTTQVERNACLFCKARKLDDKFYQKLRGQFPDAVFWQEIGEIFRQLQKQATEIYNQSLIELYYEIFIKGKGFANASSVEHYLSDVCYTRAAELFKNAAIASGLRGKVKSNFRLKELKNMKSGLPTTKSDNFPIPLVKQKGGQYTGFEISSHNDDFIIKIPFGRWQVKEEIDKYRPWEKFDFEQVRKNPKPISLLLSIQRRKRNKGWSRDEGTEAEIRKVMNGDYQTSYIEVKRGSKIGEKSAWMLNLSIDVPKIDKGVDPSIIGGIDVGVKSPLICAINNAFSRYGISDNDLFRFNKKVFARRRILLKKNRHKRAGHGTKNKLKPITILTEKSGRFRKKLIERWACEIADFFVKNKVGTVQMENLESMKRKEDSYFNIRLRGFWPYAEMQNKIEFKLKQYGIKVRKVAPNNTSKTCSKCGHLNNHFSFEYRKKNKFPHFKCEKCNFKENADYNAALNISNPKLKSTKEEP

SEQ ID NO: 2183 - protein, 726 aa, synthetic construct
SEDEFSHEYWMRHALTLAKRARDEREVPVGAVLVLNNRVIGEGWNRAIGLHDPTAHAEIMALRQGGLVMQNYRLTDATLYVTFEPCVMCAGAMIHSRIGRVVFGVRNNKHGAAGSLVNVLNYPGMNHRVEITEGILADECAALLCDFYRMPRQVFNARKKAQSSISPGGSSGGSRGSETPGTSESATPESSGGSSGGSAKNTITKTLKLRIVRPYNSAEVEKIVADEKNNREKIALEKNKDKVKEACSRHLKVAAYCTTQVERNACLFCKARRLDDKFYQKLRGQFPDAVFWQEIGEIFRQLQKQAAEVYNQSLVELYYEIFIKGKGITNASRVEHYLSDVCYTRAAELFKNAAIASGLRSKVRSNFRLKELKNMKSGLPTTKSDNFPIPLVKQKGGQYTGFEISSHNSDFIIKIPFGRWQVKEEIDKYRPWEKFDFEQVRKSPKPISLLLSTQGRQKNKGWSKDEGTEAEIRRVMNGDYQTSYIEVKRGSKIGGKSTWMLNLSIDVPKIDKGVDPSIVGGIDVGVKSPLVCAINNSFSRYSICDNDLFRFNKKMFARRRILLRKNRHKRAGHGARNKLKPITVLTEKSERFRKKLIERWACEIADFFIKNKVGTVQMENLESMKRKEDSYFNIRLRGFWPYAEMQNKIEFKLKQYGIEIRKVAPNNTSKTCSKCGHLNNYFNFEYRKKNKFPHFKCEKCNFKENADYNAALNISNPKLKSTKEEP

SEQ ID NO: 2184 - protein, 726 aa, synthetic construct
SEVEFSHEYWMRHALTLAKRARDEREVPVGAILVLNNRVIGEGWNRAIGLHDPTAHAEIMALRQGGLVMQNYRLIDATLYVTFEPCVMCAGAMIHSRIGRVVFGVRNNKHGAAGSLVNVLDYPGMNHRVEITEGILADECAALLCDFYRMPRQVFNARKKAQSSNSPGGSSGGSSGSETPGISESATPESSGGSSGGSAKNTITKTLQLRIVRPYNSAEVEKIVTDEKNNREKIALEKNKDKVKEACSKHLKMASYCTTQVERNACLFCKARKLDDKFYQKLRGQFPDAVFWQELGEIFRQLQKQAAEIYNQSLIELYYEIFIKGRGFANASSVEHYLSDVCYTRAAELFKNAAIASGLRGKVKSNFRLKELRNMKSGLPTTKSDNFPIPLVKQKGGQYTGFEISSHNDDFIIKIPFGRWQVKEEIDKYRPWEKFDFEQVRKNPKPISLLLSIQRRKRNKGWSRDEGTEAEIRKVMNGDYQTSYIEVKRGSKIGEKSAWMLNLSIDVPRIDKGVDPSIIGGIDVGVKSPLICAINNAFSRYGISDNDLFRFNKKVFARRRILLKKNRHKRAGHGTKNKLKPITILTEKSGRFRKKLIERWACEIANFFIKNKVGTVQMEDLESMKRKEDSYFNIRLRGFWPYAEMQNKIEFKLKQYGIKIRKVAPNNTSKTCSKCGHLNNYFSFEYRKKNKFPHFKCEKCNFKEDADYNAALNISNPKLKSTKEEP

SEQ ID NO: 2185 - protein, 726 aa, synthetic construct
SEVEFSHEYWMRHALTLAKRARDEREVPVGAVLVLNNRVVGVGWNRAIGLHDPTAHAEIMALRQGGLVMQNYRLTDATLYVTFEPCVMCAGAMVHSRIGRVVFGVRNSKRGAAGSLMNVLNYPGMSHCVEITEGILVDECAALLCDFYRMPRQVLNAQKKAQPSISSGGSSGGSSGSGTPSASGSVTPKSSVGSSAGSAKNTITKTLKLRIVRPYNSAEVEKIVADEKNSREKIALEKNKDKVKEACSEHLKVAAYCTTQVERNACLFCKARKLDDKFYQRLRGQFPDAVFWQEIGEIFRQLQKQAAEIYNQSLIELYYEIFIKGKGFANASSVEHYLSDVCYTRAAELFKNAAIASGLRGKVKSNFRLKELKNMKSGLPTTKSDNFPIPLVKQKGGQYTGFEINSHNDDFVIKIPFGRWRVKKEIDKYRPWEKFDFEQVRKSPKPISLLLSTQRRKRNKGWSKDEGTEAEIRKVMNGDYQTSYIEVKRGSKIGEKSAWMLNLSIGVPKIDKGVDPSIIGGIDVGVKSPLVCAINNAFSRYSISDNDLFHFNKKMFARRRILLKKNRHKRAGHGAKNKLKPISILTERSKRFRKKLIERWACEIADFFIKNKVGTVQMENLESMKRKEDSYFNIRLRGFWPYAEMQNKIEFKLKQYGIVVRKVAPNNTSKTCSKCGHLNNYFNFEYRKKNKFPHFKCEKCNFKEDADYNAALNISNPKLKSTKGEP

SEQ ID NO: 2186 - protein, 725 aa, synthetic construct
SEVEFSHEYWMRHALTLAKRARDEREVPVGAILVLNNRVIGEGWNRAIGLHDPTAHAEIMALRQGGLVMQNYRLIDATLYVTFEPCVMCAGAMIHSRIGRVVFGVRNNKHGAAGSLVNVLNYPGMNHRVEITEGILADECAALLCDFYRMPRQVFNARKKARSNIDSGCSSGGSSGSETPGTSESATPESSGGSSGGSTKNTITKTLKLRIVRPYNSAEVEKIVADEKNNREIALEKNKDKVKEACSKHLKVAAYCTTQVERNACLFCRARRLDDRFYQKLRGQFPDAVFWQETGEIFRQLQRQAAEIYNQSLIELYYEIFIKGKGFANASSVEHYLSDVCYTRAAELFKNAAIASGLRGKVKSNFRLKELKNMKSGLPTTKSDNFPIPLVKQKGGQYTGFEISSHNDDFIIKIPFGRWQVKKEIDKYRPWEKFDFEQVRKSPKPISLLLSTRRRKRNKGWSKDEGTEAEIRKVMNGDYQTSYIEVKRGSKIGEKSAWMLNLSIDVPRIDKGVDPSIIGGIDVGVKSPLVCAINNAFSRYSISDNDLFHFNKKMFARRRILLKKNRRRRAGHGAKNKLKPITILTEKSVRFRKKLIERWACEIADFFIKNKVGTVQMENLESMKRKEDSYFNIRLRGFWPYAEMQNKIEFKLKQYGIEIRRVAPNNTSRTCSKCGHLNNYFNFEYRRKYKFPHFKCEKCNFKEDADYNAALNISNPKLKSTKGEP

SEQ ID NO: 2187 - protein, 726 aa, synthetic construct
SEVEFSHEYWMRHALTLAKRARDEREVPVGAVLVLNNRVIGEGWNRAIGLHDPTAHAEIMALRQGGLVMQNYRLVDATLYVTFEPCVLCAGAMVHSRIGRVVFGVRNSKRGAAGSLMNVLNYPGMNHRVEITEGILADECAALLCDFYRMPRQVFNARKKARSNINSSGSSGGSSGSETPGTSESATPESSGGSSGGSAKNTITKTLKLRIVRPYNSAEVEKIVADEKNNREKIALEKNKDKVKEACSEHLKVAAYCTTQVERNACLFCKARKLDDKFYQKLRGQFPDAVFWQETGEIFRQLQRQAAEIYNQSLIELYYEIFIKGKGFANASSVEHYLSDVCYARAAELFKNAAIASGLRGKVKSNFRLRELKNMKSGLPTTKSDNFPIPLVKQKGGQYTGFEISSHNDDFIIKIPFGRWQVKKEIDKYRPWEKFDFEQVRKSPKPISLLLSTQRRKRNKGWSKDEGTEAEIRKVMNGDYQTSYIEVKRGSKTGEKSAWMLNLSIDVPKIDKGVDPSIIGGIDVGVKSPLVCAINNALSRYSISDNDLFHFNKKMFARRRILLRKNRHKRAGHGARNKLRPITVLTEKSERFRKKLIERWACEIANFFIKNKVGTVQMENLESMKRREDSYFNIRLRGFWPYAEMQNKIEFKLKQYGIEIRKVAPNNTSKTCSKCGHLNNYFNFEYRKKNKFPHFKCEECNFKENADYNAALNISNPKLKSTREEP

SEQ ID NO: 2188 - protein, 726 aa, synthetic construct
SEVEFSHEYWMRHALTLAKRARDEREVPVGAVLVLNNRVIGEGWNRTTGLHDPTAHAEIMALRQGGLVMQNHRLVDATLYVTFEPCVMCAGAMIHSRIGRVVFGVRNSKRGAAGSLTNVLNYPGMNHCVEITEGILADECAALLCDFYCMPRQVFNAQKRAQSSINSGGSSGGSSASETPGTSESATPESSGGGSSGSAKNTITKTLQLRIVRPYNSAEVEKIVADEKNNREKIALKKNKDKVKEACSKHLKVASYCTTQVERNACPFCKARKLDDKFYQKLRGQFPDAVFWQELGEILRQLQKQAAEIYNQSLIELYYEIFIKGRGFANASSVEHYLSDVCYTRAAELFKNAAIASGLRGKVKSNFRLKELKNMRSGLPTTKSDNFPIPLVKQKGGQYTGFEISSRNDDFIIKIPFGRWQAKKEIDRYRPWEKFDFEQVRKSPKPISLLLSTRRRKGNKGWSKDEGTEAEIRRVMNGDYQTSYIEVKRGSKIGEKSAWMLSLSIDVPKIDKGVDPRIIGGIDVGVKSPLVCAINNVLSRYSISDNDLFHFNKKMFARRRILLKKNGHKRAGHGAKNKLKPITIMTEKSKRFRKKLIERWACEIADFFIKNKVGTVQMENLESMKRKEDSYFNIRLRGFWPYAEMQNKIEFKLKQYGIEIRKVAPNNTSKTCSKCGHLNNYFNFEYRRKNKFPHFKCEKCNFKEDADYNAALNISNPKLKSTKEEP

SEQ ID NO: 2189 - protein, 726 aa, synthetic construct
SEDEFSHEYWMRHALTLAKRARDGREVPVGAVLVLNNRVIGEGWNRAIGLHDPTAHAEIMALRQGGLVMQNYRLIDATLYVTFEPCVMCAGAMVHSRIGRVVFGVRNSKRGAAGSLMNVLDYPGMGHRVEITEGILADECAALLCDFYRMPRQVFNAQKRAQSSINSGGSSGGSSGSETPGTSESATPESSGGGSSGSAKNTFTKTLQLRIVRPYNSAEVEKIVADEKDNREKIALEKNKDKVREACSRHLKVASYCTTQVERNACTFCKARKLDDKFYQKLRGQFPDAVFWQELGEILRQLQKQAAEIYNQSLIELYYEIFIKGRGFANASSVEHYLSDVCYTRAAELFKNAAIASGLRGKVKSNFRLKELKNMKSGLPTTKSDNFPIPLVKQKGGQYTGFEISSHNDDFIIKIPFGRWQVKKEIDKYRPWEKFDFEQVRKSPKPISLLLSTQRRKRNKGWSKDEGTEAEIRKVMNGDYQTSYIEVKRGSKVGEKSAWMLNLSIDVPKIDKGVDPSITGGIDVGVKSPLVCAINNALSRYSISDNDLFHFNKKMFARRRILLRKNRHKRAGHGARNKLKPITVLTEKSERFRKKLIERWACEIANFFIKNKVGTVQMENLESMKRREDSYFNIRLRGFWPYAEMQNKIEFKLKQYGIEIRKVAPNNTSKTCSKCGHLNNYFNFEFRKKNKFPHFKCEKCNFKENADYNAALNISNPKLKSTKEEP

SEQ ID NO: 2190 - protein, 726 aa, synthetic construct
SEDEFSHEYWMRHALTLAKRARDGREVPVGAVLVLNNRVIGEGWNRAIGLHDPTAHAEIMALRQGGLVMQNYRLIDATLYVTFEPCVMCAGAMVHSRIGRVVFGVRNSKRGAAGSLMNVLDYPGMGHRVEITEGILADECAALLCDFYCMPRQVFNAQKRAQSSINSGGSSGGSSGSETPGTNESATPESSGGGSGGSAKNTITKTLTLRIVRPYNSAEVEKIVADEKNNREKIALEKNKDKVKEACSKHLKVAAYCTTQVERNACLFCKARKLDDKFYQKLRGQFPEAVFWQELGEIFRQLQKQAAEIYNQSLIELYYEIFIKGKGFANASSVEHYLSDVCYTRAAELFKNAAIASGLRGKVKSNFRLKELKNMKSGLPTTKSDNFPIPLVKQKGGQYTGFEISSHNDDFIIKIPFGRWQVRKEIDKYRPWEKFNFEQVRKSPKPISLLLSTQRRKRNKGWSKDEGTEAEIRKVMNGDYQTSYIEVKRGSKIGEKSAWMLNLSIDVPKIDKGVDPGIIGGIDVGVKSPLVCAINNASSRYSISDNDLFHFNKKMFARRRILLKKNRHKRAGHGAKNKLKPITILTEKSERFRKKLIERWACEVADFFIKNRVGTVQMENLEGMKRKEDSYFNIRLRGFWPYAEMQNRIEFKLKQYGIEIRRVAPNNTSRTCSKCGHLNNYFNFEYRKKNKFPHFKCEKCNFREDADYNAALNISNPKLKSTKEEP

SEQ ID NO: 2191 - protein, 726 aa, synthetic construct
SEVEFSHEYWMRRALTLAKRARDEREVPVGAVLVLNNRVIGVGWNRAVGLHDPTAHAEIMALRQGGLVMQNYRLVEATLYVTFEPCIMCAGAMIHSRIGRVVFGVRNSKRGAAGSLMNVLNYPGMNHRVEITEGILADECAALLCDYYRMPRQVFNARKKAQSSINSGGSSDGGSGSETPGTSESATPESSGGSSGGSAKNTITKTLKLRIVRPYNSAEVEKIVADEKNNREKIALEKNKDKVKEACSKHLKVAAYCTTQVERNACLFCKARKLDDKFYQKLRGQFPDAVFWQEIGEIFRQLQKQAAEIYNQSLIELYYEIFIKGKGFANASSVEHYLSDVSYTRAAELFKNAAIASGLRGKVKSNFRLKELKNMKSGLPTTKSDNFPIPLVKQKGGQYTGFEISSHNDDFIIKIPFGRWQVKEEIDKYRPWEKFDFEQVRKNPKPISLLLSTQRRKGNKGWSKDEGTEAEIRKVMNGDYQTSYIEVKRGNKIGEESAWMLNLSIDVPKIDKGVDPSIIGGIDVGVKSPLVCAINNALSRYSISDNDLFRFNKKMFARRRILLKKNRHKRAGHGVKNKLKPITILTEKSGRFRKKLIERWACEIADFFVKNKVGTVQIENLESMKRKEDSYFNIRLRGFWPYAEMQNKIEFKLKQYGIKVRKVAPNNTSKTCSKCGHLNNYFSFEYRKKNKFPHFKCEKCNFKENADYNAALNISNPKLKSTKEEP

SEQ ID NO: 2192 - protein, 726 aa, synthetic construct
SEVEFSHEYWMRHALTLAKRARDEREVPVGAVLVLNNRVIGEGWNRAIGLHDPTAHAEIMALRQGGLVMQNYRLTDATLYVTFEPCVMCAGAMIHSRIGRVVFGVRNSKRGAAGSLMNVLNYPGMNHCVEITEGILVDECAALLCDFYRMPRQVLNAQKKAQPSINSGGSSGGGSGSETPSTSESTTPESSGGSSGGSAKNTITKTLKLRIVRPYNSAEVEKIVADEKNNREKVALERNKDKVKEACSKHLKVASYCTTQVERNACPFCKARKLDDKFYQKLRGQFPDAVFWQEIGEIFRQLQKQAAEIYNQSLIELYYEIFIKGRGFANASSVEHYLSDVCYTRAAELFKNAAIASGLRGKVKSNFRLKELKNMRSGLPTTKSDNFPIPLVKQKGGQYAGFEISNHNGDFIIKIPFGRWQVKKEICKHRPWEKFDFEQVRKSPKPISLLLSTQRRKRNKGWGKDEGTEAEIRKVMNGDYQTSYIEVKRGSKIGEKSAWMLNLSIDVPKIVKGVDPSIIGGIDVGVKSPLVCAINNAFSRYSISDNDLFHFNKKMFARRRILLKKNRHKRAGHGAKNKLKPISILTEKSKRFRKKLIERWACEIADFFIKNKVGTVQMENLEGMRRKEDSYFNIRLRGFWPYAEMQNKIEFKLKQYGIEIRKVAPNNTSKTCSKCGHLNHYFNFEYRKKNKFPHFRCEKCNFKENADYNAALNISNPKLKSTKEEP

SEQ ID NO: 2193 - protein, 726 aa, synthetic construct; identical to SEQ ID NO: 684

SEQ ID NO: 2194 - protein, 726 aa, synthetic construct
SEVEFSHEYWMRHALTLAKRARDVREVPVGAVLVLNNRVIGEGWNRAIGLHDPTAHAEIMALRQGGLVMQNYRLVNATLYVTFEPCVMCAGAMIHSRIGRVVFGVRNSKRGAAGSLMNVLNYPGMNHRVEITEGILTDECAALLCDFYRMPHQVLSAQKKAQSSINSGGSSGGSSGSETPGTSGSATPESSGGSSGGSAKNTITKTLKLRIVRPYNSAEVEKIVADEKNNREKTALEKNKDKVKEACGKHLKVAAYCTTQVERNACLFCKARKLDDKFYQKLRGQFPDAVFWRETGEIFRQLQRQAAEIYNQSLIELYYEIFIKGKGFANASSVEHYLSDVCYTRAAELFKNAAIASGLRGKVKSNFRLKELKNMKSGLPTTKSDNFPIPLVKQKGGQYTGFEISSHNDDFIIKIPFGRWQVKKEIDRYRPWEKFDFEQVRKSPKPISLLLSTQRRKRNKGWSKDEGTEAEIRKVMNGDYQTSYIEVKRGSKIGEKSAWMLNLSIDVPKIDKGVDPSIIGGIDVGVKSPLVCAINNALSRYSISDNDLFHFNKKMFARRRILLRKNRHKRAGHGAKNKLKPITMMTEKSKRFRKKLIERWACEIADFFIKNKVGTVQMENLESMKRKEDSYFNIRLRGFWPYAEMQNKIEFKLKQYGIVVRKVAPNNTSKTCSKCGHLNNYFNFEYRKKNKFPHFKCEKCNFKEDADYNAALNISNPKLKSTKGEP

SEQ ID NO: 2195 - protein, 726 aa, synthetic construct
SEVEFSHEYWMRHALTLAKRARDEREVPVGAVLVLNNRVIGEGWNRAIGLHDPTAHAEIMALRQGGLVMQNYRLTDATLYVTFEPCVMCAGAMIHSRIGRVVFGVRNSKRGAAGSLMNVLNYPGMNHCVEITEGILVDECAALLCDFYRMPRQVFNARKKAQSSTNSGGSSDGGSGCETPGTSESATPESSGGSSGGSAKNTITKTLKLRIVRPYNSAEVEKIVADEKSNREKIALEKNKDKVKEACSKHLKVAAYCTTQVERNACLFCRARRLDDKFYQKLRGQFPDAVFWQEIGEIFRQLQKQAAEVYNQSLVELYYEILIKGKGIANASSVEHYLSNVCYTRAAELFKNAAIASGLRNKIKSNFRLKELRNMKSGLPTTKSDNFPIPLVKQKGGQYTGFEISSHNDDFIIKIPFGRWQVKKEIDKYRPWEKFDFEQVRKSPKPISLLLSTQRRQKNKGWSKDEGTEAEIRRVMNGDYQTSYIEVKGGGKIGEKSTWMLNLSIDVPKIDKGVDPSIVGGIDVGVKSPLVCAINNSFSRYSICDNDLFRFNKKMFARRRILLKKNRHKRAGHGAKNKLKPISILTGKSERFRKKLIERWACEIADFFIKNKVGTVQMENLESMKRKEDSYFNIRLRGFWPYAEMQNKIEFKLRQYGIEVRKVAPNNTSKTCSKCGHLNNYFNFEYRRKNKFPHFKCEKCNFKENADYNAALNISNPKLKSTKEEP

SEQ ID NO: 2196 - protein, 726 aa, synthetic construct
SEVEFSHEYWMRHALTLAKRARDEREVPVGAVLVLNNRVIGEGWNRAIGLHDPTAHAEIMALRQGGLVMQNYRLVDATLYVTFEPCVLCAGAMVHSRIGRVVFGVRNSKRGAAGSLMNVLNYPGMNHRVEVTEGILADECAALLCDFYRMPRQVFNAQKKARSNINSGGSSGGSSGSEMPGTSESATPESSGGSSGGSAKNTITKTLKLRIVRPYNSAEVEKIVADEKNNREKIALEKNKDKVKEACSEHLKVAAYCTTQVERNACLFCKARKLDDKFYQKLRGQFPDAVFWQEVSEIFRQLQKQAAVIYNQSLIELYYEIFIKGKGFANASSVEHYLSDVCYTRAAELFRNAAIASGLRGKVKSNFRLKELKNMKSGLPTTKSDNFPIPLVKQKGGQYTGFEISNHNDDLIIKIPFGRWQVKKEIDKYRPWEKFDFEQVRKSPKPISLLLSTQRRKRNKGWSKDEGTEAEIRRVMNGDYQISYIEVKRGSKIGEKSAWMLNLSIDVPKIDKGVDPSIVGGIDVGVKSPLVCAINNAFSRYSISDNDLFHFNKKMFARRRILLKKTRHKRAGHGAKNKLKPISILTEKSERFRKKLIERWACEIADFFIKNKVGTVQMENLESMKRREDSYFNIRLRGFWPYAKMQNKIEFKLKQYGIEIRKVAPNNTSKTCSKCGHLNDYFNFEYRKKNKFPHFKCEKCNFKESADYNAALNISNPKLKSTKEEP

SEQ ID NO: 2197 - protein, 726 aa, synthetic construct
SEVEFSHEYWMRHALTLAKRARDEREVPVGAVLVLNNRVIGEGWNRAIGLHDPTAHAEIMALRQGGLVLQNYRLVDATLYVTFEPCVLCAGAMVHSRIGRVVFGARNSKRGAAGSLMNILNYPGMNHRVEITEGILADECAALLCDFYRMPRQVFNAQKKAQSSINSGGSSGGSSGSETPSTSECATPESSGGSSGGSAKNTTTKTLQLRIVRPYNSAEVEKIVTDEKNNREKIALEKNKDKVKEACSKHLKMASYCTTQVERNACLFCKARKLDDKFYQKLRGQFPDAVFWQELGGIFRQLQKQAAEIYNQSLIELYYEIFIKGKGITNASRVEHYLSDVCYTRAAELFKNAAIASGLRSKVRSNFRLKELKNMKSGLPTTKSDNFPIPLVKQKGGQYTGFEISNHNSDFIIKIPFGRWRVKEEIDKYRPWEKFDFEQVRKSPKPISLLLSTQRRKKNKGWSKDEGTEAEIRRVMNGDYQTSYIEVKRGSKIGEKSAWMLNLSIDVPKIDKGVDPSIIGGIDVGVKSPLVCAINNAFSRYSISDNDLFHFNKKMFARRRILLKKNGRKRVGHGAKNKLKPITILTEKSKRFRKKLIERWACEIAGFFIKNKVGTVQMENLESMKRKEDSYFNIRLRGFWPYAEMQNKIEFKLKQYGIEIRKVAPDNTSKTCSMCGHLNNYFNFEYRKKNKFPHFKCEKCNFKEDADYNAALNISNPKLKSTKEEP

SEQ ID NO: 2198 - protein, 726 aa, synthetic construct
SEVEFSHEYWMRHALTLAKRARDEREVPVGAVLVLNNRVIGEGWNRTTGLHDPTAHAEIMALRQGGLVMQNHRLVDATLYVTFEPCVMCAGAMIHSRIGRVVFGVRNSKRGAAGSLTNVLNYPGMNHRVEITEGILVDECAALLCDFYRMPRQVFSAQKKAQSTINSGGSSGGSSGSETPGTSESPTPESSGGSPGGSAKNTITKTLKLRIVRPYNSAEVEKIVADEKNNREKIALEKNKDKVKEACSKHLKVASYCTTQVERNACLFCKARKLDDKFYQKLRGQFPDAVFWQELGEIFRQLQKQAAEIYNQSLIELYYEIFIKGKGLANASSVEHYLSDVCYTRAAELFKNAAIASGLRGKVKSNFRLKELKSMKSGLPSTKSDNFPIPLVKQKGGQYTGFEISSHNSDFIIKIPFGRWQVKEEIDKYRPWEKFDFEQVRKSPKPISLLLSTQRRKKNKGWSKDEGTEAEIRRVMNGDYQTSYIEVKRGSKIGEKSAWMLNLSIDVPTIDKGVDPSIIGGIDVGVKSPLVCAINNASSRFSISDNDLFHFNKKMFARRRILLKKNGRKRAGHGAKNKLKPITILTEKSKRFRKKLIERWACEIAGFFIKNKVGTVQMENLESMKRKEDSYFNIRLRGFWPYAEMQNKIEFKLKQYGIEIRKVAPNNTSKTCSKCGHLNDYFNFEYRKKNKFPHFKCEKCNFKENADYNAALNISSPKLKSTREEP

SEQ ID NO: 2199 - protein, 726 aa, synthetic construct
SEVEFSHEYWMRHALTLAKRARDEREVPVGAVLVLNNRVIGEGWNRAIGLHDPTAHAEVMALRQGGLVMQNYRLTDATLYVTFEPCVMCAGAMIHGRIGRVVFGVRNSKRGAAGSLMNVLNYPGMNHRVEITEGILADECAALICDYYRMPRQVFNARKKAQSSINSGGSSDGGSGSETPGTSESATQESSGDSSGGSAKNTITKTLKLRIVRPYNSAEVEKIVADEKNNREKIALERNKDKVKEACSEHLKVAAYCTTQVERSACLFCKARKLDDKFYQKLRGQFPDAVSWQEIGEIFRQLQKQAAEIYNQSLIELYYEIFIKGKGFANASSVEHYLSDVCYTRAAELFKNAAIASGLRGKVKSNFRLKELKNMKSGLPTTKSDNFPIPLVKQKGGQYTGFEISSHNGDFIIKIPFGRWQVKKEIDKYRPWEKFDFEQVRKSPKPISLLLSTQRRKRNKGWSKDEGTEAEIRKVMNGDYQTSYIEVKRGSKIGEKSVWMLNLSIDVPKIDKGVDPCIIGGIDVGVKSPLVCAINNAFSRYSISDNDLFHFNKKMFARRRILLKENGHKRAGHGAKNKLKPLTIMTEKSKRFRKKLIERWACEIADFFIKNKVGTVQMENLESMKRKEDSYFNIRLRGFWPYAEMQNKIEFKLKQYGIVVRKVAPNNTSKTCSECGHLNNYFNFEYRKKNKFPHFKCEKCNFKENADYNAALNISNPKLKSTKGEP

SEQ ID NO: 2200 - protein, 726 aa, synthetic construct
SEVEFSHEYWMRHALTLAKRARDEREVPVGAVLVLNNRVIGEGWNRAIGLHDPTAHAEIMALRQGGLVMQNYRLTGATLYVTFEPCVMCAGAMIHSRIGRVVFGVRNSKRGAAGSLMNVLNYPGMDHCVEITEGILVDECAALLCDFYRMPRQVLNAQKKAQSSISSGGSSGGSSGSVTPGASGSVTPKSSGGSSAGSTKDTITKTLKLRIVRPYNSAEVEKIVADEKNNREKIAMEKNKDKVKEACSKHLKVATYCTTQVERNACLFCKARKLDDKFYQELRGQFPDAVFWQEIGEIFRQLQKQAAEIYNQSLIELYYEIFIKGKGFANAGSVEHYLSDVCYTRAAGLFKNAAIASGLRGKVKSNFRLKELKNMKSGLPTTKSDNFPIPLVKQKGGQYTGFEISSHNDDFIIKIPFGRWQAKKEIDKYRPWEKFDFEQVRKSPKPISLLLSTQRRKRNRGWSKDEGTEAEIRKVMNGDYQTSYIEVKRGSKIGEKSAWMLNLSIDVPKIDKGVDPSIIGGIDVGVKSPLVCAINNAFSRYSISDNDLFRFNKKMFARRRILLKKNRHKRAGHGAKNKLKPITILTEKSGRFRKKLIERWACEIADFFIKNKVGTVQMENLESMKRREDSYFNIRLRGFWPYAKMQNKIEFKLKQYGIKVRKVAPNNTSKTCSKCGHLNNYFSFEYRKKNKFPHFKCEKCNFKENADYNAALNISNPKLKSTKEEP

SEQ ID NO: 2201 - protein, 725 aa, synthetic construct
SEVEFSHEYWMRHALTLAKRARDEREVPVGAVLVLNNRVIGEGWNRAIGLHDPTAHAEIMALRQGGLVMQNYRLIDATLYVTFEPCVMCAGAMVHSRIGRVVFGVRNSKRGAAGSLMNVLDYPGMGHRVEITEGILADECAALLCDFYCMPRQVFNAQKRAQSSINPGGSSGGSSGSETPGTSESASPESSGGGSSGSAKNTITKTLQLRIVRPYNSAEVEKIVADEKNNREKIALEKNKDKVKEACSEHLKVATYCTTRVERNACPFCRARKLDDKFYQKLRGQFPDAVFWQELGEIFRQLQKQAAEIYNQSLIELYYEIFIKGKGFANASSVEHYLSDVCYTRAAELFKNAAIASGLRGKVKSNFRLKELKNMKSGLPTTKSDNFPIPLVKQKGGQYTGFEISSHNDDFIIKIPFGRWVKKEIDKYRPWEKFDFEQVRRSPKPISLLLSTQRRKRNKGWSKDEGTEAEIRKVMNGDYQTSYIEVKRGSKIGEKSAWMLNLSIDVPKIDKGVDPSIIGGIDVGVKSPLVCAINNALSRYSISDNDLFHFNKKMFARRRILLRKNRHKRAGHGAKNKLKPITIMTEKSKRFRKKLIERWACEIADFFIKNKVGTVQMENLESMKRKEDSYFNIRLRGFWPYAEMQNKIEFKLKQYGIGIRKVTPNNTSKTCSKCGHLNNYFNFEYRKKNKFPHFKCEKCNFKENADYNAALNISNPKLKSTKEEP

SEQ ID NO: 2202 - protein, 726 aa, synthetic construct; identical to SEQ ID NO: 684

SEQ ID NO: 2203 - protein, 726 aa, synthetic construct; identical to SEQ ID NO: 684

SEQ ID NO: 2204 - protein, 726 aa, synthetic construct
SEAEFSHEYWMRHALTLAERARDEREVPVGAILVLNNRVIGEGWNRAIGLHDPTAHAEIMALRQGGLVMQNYRLIDATLYVTFEPCVMCAGAMIHSRIGRVVFGVRNNKHGAAGSLVNVLNYPGMNHRVEITEGILADECAALLCDFYRMPRQVFNARKKAQSSINPGGSSGGSSGNETPGTSESATPESSGGSSGSSAKNTITKTLKLRIVRPYNSAEVEKIVADEKSNREKIALEKNKDKVKEACSKHLKVAAYCTTQVERNACLFCKARRLDDKFYQKLRGQFPDAVFWQEIGEIFRQLQRQAAEIYNRSLIELYYEIFIKGKGFANASSVEHYLSDVCYTRAAELFKNAAIASGLRGKVKSNFRLKELKNMKSGLPTTKSDNFPIPLVKQKGGQYTGFEISSHNDDFIIKIPFGRWQAKKEIDKYRPWEKFDFEQVRKSPKPISLLLSTQRRKRNKGWSKDEGTEAEIRKVMNGDYQTSYIEVKRGSKIGEKSAWMLSLSIDVPKIDKGVDPSIIGGIDVGVKSPLVCAINNAFCRYSISDNDLFHFNKKMFARRRILLKKSRHKRAGHGAKNKLKPISILTEKSERFRKKLIERWACEIANFFIKNKVGTVQMENLESMKRKEDSYFNIRLRGFWPYAEMQNKIEFKLKQYGIKIRKVAPNNTSKTCSKCGHLNNYFNFEYRKKNKFPHFKCEKCNFKEDADYNAALNISNPKLKSTKEEP

SEQ ID NO: 2205 - protein, 726 aa, synthetic construct; identical to SEQ ID NO: 684

SEQ ID NO: 2206 - protein, 726 aa, synthetic construct
SEVEFSHEYWMRHALTLAKRARDEREVPVGAILVLNNRVIGEGWNRAIGLHDPTAHAEIMALRQGGLVMQNCRLVDATLYVTFEPCVMCAGAMIHSRIGRVVFGVRNSKRGAAGSLMNVLNYPGMNHRVEITEGILAGECAALLCDFYRMPRQVFNAQKKAQSTINSGGSSGGSSSSETPGISGSATPEGSGGSSGGSAKNTITKTLKLRIVRPYNSAEVEKIVADEKNNREKIALEKNKDKVKEACSKHLKVASYCTTQVERNACLFCKARKLDDKFYQKLRGQFPDAVFWQELGEIFRQLQKQAAEIYNQSLIELYYEIFIKGKGFANASSVEHYLSDVCYTRAAELFKNAAIASGLRGKVKSNFRLKELKNMKSGLPTTKSDNFPIPLVKQKGGQYTGFEISNHNSDFIIKIPFGRWQAKKEIDKYRPWEKFDFEQVRKSPKPISLLLSTQRRKKNRGWSKDEGTEAEIKKVLNGDYQTSYIEVKRGSKIGEKSAWMLNLSIDVPKIDKGVDPSIIGGIDVGVKSPLVCAISNAFSRYSISDNDLFHFNKKMFARRRILLKKSKHKRAGHGAKNKLKPITILTEKSRRFRKKLIERWACEIADFFIKNKVGTVQMENLESMKRREDSYFNIRLRGFWPYAEMQNKIEFKLKQYGIEIRKVAPNNTSKTCSKCGHLNNYFNFEYRKKNKFPPFKCEKCNFKENADYNAALNISNPKLKSTKEEP

SEQ ID NO: 2207 - protein, 726 aa, synthetic construct; identical to SEQ ID NO: 684

SEQ ID NO: 2208 - protein, 726 aa, synthetic construct; identical to SEQ ID NO: 684

SEQ ID NO: 2209 - protein, 726 aa, synthetic construct
SEVEFSHEYWMRHALTLAKRARDEREVPVGAVLVLNNRVIGEGWNRAIGLHDPTAHAEIMALRQGGLAMQNYRLVDATLYVTFEPCVLCAGAMVHSRIGRVVFGVRNSKRGAAGSLMNVLNHPGMDHRVEITGGILADECAALLCDFYRMPRRVFNAQKKAQSSINSGGSSGGSSGSVTPGTSESATPESSGGSFGGSAKNTITKTLQLRIVRPYNSAEVEKIVADEKNNREKIALEKNKDKVKEACSKHLKVAPYCTTQVERNACPFCKARKLDDKFYQKLRGQFPDAVFWQELGEIFRQLQKQAAEIYNQSLIELYYEIFIKGKGFANASSVEHYLSDVCYTRAAELFKNAAIASGLRGKVKSNFRLKELKNMKSGLPTTKSDNFPVPLVKQKGGQYTGFEISNHNSDFIIKIPFGRWQVKEEINKYRPWEKFDFEQVRKSPKPISLLLSTQRRKRNKGWSKDEGTEAEIRKVMNGDYQTSYIEVKRGSKIGEKSAWMLSLSIDVPKIDKGVDPSIIGGIDVGVKSPLVCAINNAFCRYSISDNDLFHFNKKMFARRRILLKKSRHKRAGHGAKNKLKPISILTEKSGRFRKKLIERWACEIANFFIKNRVGTVQMENLESMKRKEDSYFNIRLRGFWPYAEMQNKIEFKLKQYGIKIRKVAPNDTSKTCSKCGHLNNYFSFEYRKKNKFPHFKCEKCNFKEDADYNAALNISNPKLKSTKEEP

SEQ ID NO: 2210 - protein, 726 aa, synthetic construct; identical to SEQ ID NO: 684

SEQ ID NO: 2211 - protein, 726 aa, synthetic construct
SEVEFSHEYWMRHALTLAKRARDEREVPVGAILVLNNRVIGEGWNRAIGLHDPTAHAEVMALRQGGLVMQNYRLIDATLYVTFEPCVMCAGAMVHSRIGRVVFGVRNSKRGAAGSLMNVLDYPGMDHRVEITEGILVDECAALLCDFYRMPRQVFNAQKKAQSSINSGGSSGGSSGSVTPGASGSVTPKSSGGSSAGSTKDTITKTLQLRIVRPYNSAEVEKIVADEKNNREKIALEKNKDKVKEACSKHLKVASYCTTQVERNACPFCKARKLDDKFYQKLRGQFPDAVFWQELGEILRQLQKQAAEIYNQSLIELYYEIFIKGKGFANASSVEHYLSDVCYTRAAELFKNAAIASGLRGKVKSNFRLKELKNMKSSLPTTKSDNFPIPLVKQKGGQYTGFEISSHNDDFIIKIPFGRWQVKKEIDKYRPWEKFVFEQVRKSPKPISLLLSTQRRKRNKGWSKDDGTEAEIRKVMNGDYQTSYIEVKRGSKIGEKSAWMLNLSIDVPKIDKGVDPSIIGGIDVGVKSPLVCAINNAFSRYSISDNDLFRFNKKMFARRRILLGKNRHKRAGHGVKNKLKPITILTEKSGRFRKKLIERWACEIADFFVKNKVGTVQMENLESMKRKEDSYFNIRLRGFWPYAEMQNKIEFKLKQYGIKVRKVAPNNTSKTCSKCGHLSNYFSFEYRKKNKFPHFKCEKCNFKENADYNAALNISNPKLKSTKEEP

SEQ ID NO: 2212 - protein, 726 aa, synthetic construct
SEDEFSHEYWMRHALTLAKRARDGREVPVGAVLVLNNRVIGEGWNRAIGLHDPTAHAEIMALRQGGLVMQNYRLIDATLYVTFEPCVMCAGAMVHSRIGRVVFGVRNSKRGAAGSLMNVLDYPGMGHRVEITEGILADECAALLCDFYRMPCQVFNAQKRAQSSINSGGSSGGSSGSDTPGTSESATPESSGGGSSGSAKNTITKTLQLRIVRPYNSAEVEKIVADEKNNREKIALEKNKEKVKEACSKHLKVASYCTTQVERNACPFCKARKLDDKFYQKLRGQFPDAVFWQELGEILRQLQKQAAEIYNQSLIELYYEIFIKGKGFANASSVEHYLSDVCYTRAAELFKNAAIASGLRGKVKGNFRLKELKNMKSGLPTTKSDNFPIPLVKQKGGQYTGFEISSHNDDFIIKIPFGRWQVKKEINKFRPWEKFDFEQVRKSPKPISLLLSTQRRKRNKGWSRDEGTEAEIRKVMNGDYQTSYIEVKRGSKIGEKSAWMLSLSIDVPKIDKGVDPSIIGGIDVGVKSPLVCAINNAFGRYSISDNDLFHFNKKMFAMRRILLKKNRHKRAGHGAKNKLKPITILTEKSKRFRKKLIERWACEIADFFIKNKVGTVQMENLESMKRKEDSYFNIRLRGFWPYAEMQDKIEFKLKQYGIEIRKVAPNNTSKTCSRCGHLNNYFNFEYRRKNKFPHFKCEKCNFKENADYNAALNISNPKLKSTKEEP

SEQ ID NO: 2213 - protein, 726 aa, synthetic construct
SEVEFSHEYWMRRALTLAKRARDEREVPVGAVLVLNNRVIGVGWNRAAGLHDPTAHAEIMALRQGGLVMQNYRLVEATLYVTFEPCIMCAGAMIHSRIGRVVFGVRNSKRGAAGSLMNVLNYPGMNHRVEITEGILADECAALLCDYYRMPRQVFNAQRKAQSTINSGGSSGGSSSSETPGTSGSATPESSGGSSGGSAKNTITKTLKLRIVRPYNSAEVEKIVADEKNNREKIALEKNKDKVKEACSKHLKVASYCTTQVERNACLFCKARKLDDKFYQKLRGQFPDAVFWQELGEIFRQLQKQAAEVYNQSLIELYYEIFIKGKGFANASSVEHYLSDVCYTRAAELFKNAAIASGLRGKVKSNFRLKELKNMKSGLPTTKSDNFPIPLVKQKGGQYTGFEISSHNDDFIIKIPFGRWQVKKEIDRYRPWEKFDFEQVRKSPKPISLLLSTQRRKRNKGWSKDEGTEAEIRKVMNGDYQASYIEVKRGSKIGEKSAWMLNLSIDVPKIDKGVDPNIIGGIDVGVKSPLVCAINSALSRYSISDNDLFHFNKKVFARRRILLGKNRHKRAGHGVKNKLKPITILTEKSGRFRKKLIERWACEIADFFVKNMVGTVQMENLESMKRKEDSYFNIRLRGFWPYAEMQNKIEFKLKQYGIKVRKVAPNNTSKTCSKCGHLNNYFSFEYRKKNKFPHFKCEKCNFKENADYNAALNISNPKLKSTKEEP

SEQ ID NO: 2214 - protein, 726 aa, synthetic construct
SEVEFSHEYWMRHALTLAKRARDEREVPVGAVLVLNNRVIGVGWNRAIGLHDPTAHAEIMALRQGGLVMQNYRLTDATLYVTFEPCVMCAGAMVHSRIGRVVFGVRNSKRGAAGSLMNVLNYPGMSHCVEITEGILVDECAALLCDFYRMPRQVLNAQKRAQSSINSGGSSDGSSGSETPGTSESATPESSGGGSSGSARNTITKTLQLRIVRPYNSAEVEKIVTDEKNNREKIALEKNKDKVKEACSKHLKMAAYCTTQVERNACLFCKARKLDDKFYQKLRGQFPDAVFWQEVGEIFRQLQKQAAEIYNQSLIELYYEIFIKGKGFANASSVEHYLSDVCYTRAAELFKNAAIASGLRGKVKSNFRLRELKNMKSGLPTTKSDNFPIPLVKQKGGQYTGFEISNHNSDFIIKIPFGRWQVKKEINKYRPWEKFDFEQVRKSPKPISLLLSTQRRKRNKGWSKDEGTEAEIRKVMNGDYQTSYIEVKRGSKTGEKSAWMLNLSIDVPKIDKGVDPSIIGGIDVGVKSPLVCAINNAFSRYSISDNDLFRFNKKMFARRRILLKKNRHKRAGHGAKNKLKPISILTGKSERFRKKLIERWACEIADFFIKNKVGTVQMENLESMKRKEDSYFNIRLRGFWPYAEMQNKIEFKLKQYGIEIRKVAPNNTSKTCSKCGHLNNYFNFEYRKKNKFPHFKCEECNFKENADYNAALNISNPKLKSTKEEP

SEQ ID NO: 2215 - protein, 726 aa, synthetic construct
SEDEFSHEYWMRHALTLAKRARDEREVPVGAILVLNNRVIGEGWNRAIGLHDPTAHAEIMALRQGGLVTQNYRLIDATLYVTFEPCVMCAGAMIHSRIGRVVFGVRNSKHGAAGSLVNVLNYPGMDHRVEITGGILADECAALLCDFYRMPRRVFNAQKKAQSSINSGGSSGGSNGSVTPGTSESATPESSGGSFGGSAKNTVTKTLQLRIVRPYNSAEVEKIVADEKNSREKIALEKNKDKVKEACSEHLKVAAYCTTQVERSACLFCKARKLDDKFYQKLRGQFPDAVFWQEIGEIFRQLQKQAAEIYNQSLIELYYEIFIKGKGFANASSVEHYLSDVCYTRAAELFKNAAIASGLRGKVKSNFRLKELKNMKSGLPTTKSDNFPIPLVKQKGGQYTGFEISSHNDDFIIKIPFGRWQVKKEINKYRPWEKFDFEQVRKGPKPISLLLSTQRRKRNKGWSKDEGTEAEIRKVMSGDYQTSYIEVKRGSKIGEKSTWMLNLSIDVPKIDKGVDPSIIGGIDVGVKSPLVCAINNAFSRYSISDNDLFRFNKKVFARRRILLKKNRHKRAGHGTKNKLKPITILTEKSGRFRKKLIERWACEIANFFIKNKVGTVQMENLESMKRKEDSYFNIRLRGFWPYAEMQNKIEFKLKQYGIEIRKVAPNNTSKTCSRCGHLNNYFSFEYRKKNKFPHFKCEKCNFKEDADYNAALNISNPKLKSTKEEP

SEQ ID NO: 2216 - protein, 726 aa, synthetic construct
SEDEFSHEYWMRHALTLAKRARDGREVPVGAVLVLNNRVIGEGWNRAIGLHDPTAHAEIMALRQGGLVMQNYRLIGATLYVTFEPCVMCAGAMVHSRIGRVVFGVRNSKRGAAGSLMNVLDYPGMGHRVEITEGILADECAALLCDFYCMPCQVFNAQKRAQSSINSGGSSGSSSGSETLGTSESATPESSGGSSAGSAKNTITKTLKLRIVRPYNSAEVEKIVADEKNNREKIALEKNKDKVKEACSEHLKVAAYCTTQVERNACLFCRARKLDDKFYQKLRGQFPDAVFWQEIGEIFRQLQKQAAEIYNQSLIELYYEIFIKGKGFANASSVEHYLSDVCYTRAAELFKNAAIASGLRGKVKSNLRLKELKNMKSGLPTTKSDNFPIPLVKQKGGQYTGFEISSHNDDFIIKIPFGRWQAKKEIDKYRPWEKFDFEQVRKSPKPISLLLSTQRRRRNRGWSKDEGTEAEIKKVMNGDYQTSYIEVKRGSKIGEKSAWMLSLSIDVPKIDKGVDPSIIGGIDVGVKSPLVCAINNAFSRYSISDNDLFHFNKKMFARRRILLKKSKHKRAGHGAKNKLKPITILTEKSGRFRKKLIERWACEIADFFIKNKVGTVQMENLESMKRKEDSYFNIRLRGFWPYAEMQNKIEFKLKQYGIEIRKVAPNNTSKTCSKCGHLNNYFNFEYRKKNKFPHFKCEKCNFKENADYNAALNISNPKLKSTKEEP

SEQ ID NO: 2217 - protein, 726 aa, synthetic construct
SEVEFSHEYWMRRALTLAKRARDEREVPVGAVLVLNNRVIGVGWNRAAGLHDPTAHAEIMALRQGGLVMQNYRLIEATLYVTFEPCIMCAGAMIHSRIGRVVFGVRNSKRGAAGSLMNVLNYPGMNHRVEITEGILADECAALLCDYYRMPRQVFNARKKVQSSINSGGSSDGGSSSETPGTIESATPESSGGSSGGSAKNTITKTLKLRIVRPYNSAEVEKIVADEKNNREKIALEKNKDRVKEACSEHLKVAAYCTTQVERNACLFCKARKLDDKFYQRLRGQFPDAVFWQELGEIFRQLQKQAAEIYNQSLIELYYEIFIKGKGFANASSVEHYLSDVCYTRAAELFKNAAIASGLRGKVKSNFRLKELKNMKSGLPTTKSDNFPIPLVRQKGGQYTGFEISSHNDDFIIKIPFGRWQVKKEIDKYRPWEKFDFEQVRKSPKPISLLLSTQRRKRNKGWSKDEGTEAEIRKVMNGDYQTSYIEVKRGSKTGGKSAWMLNLSIDVPKIDKGVDPCIIGGIDVGVKSPLVCAINDAFSRYSISDNDLFHFNKKMFARRRILLKKNGHKRAGHGAKNKLRPITIMTEKSKRFRKKLIERWACEIADFFIKNKVGTVQMENLESMKRKEDSYFNIRLRGFWPYAEMQNKIEFKLKQYGIEIRKVAPNNTSKTCSKCGHLNSYFNFEYRKKNKFPHFKCEKCNFKENADYNAALNISNPKLKGTKEEP

SEQ ID NO: 2218 - protein, 726 aa, synthetic construct
SEVEFSHEYWMRHALTLAKRARDEREVPVGAVLVLNNRVIGEGWNRAIGLHDPTAHAEIMALRQGGLVMQNYRLIDATLYVTFEPCAMCAGAMVHSRIGRVVFGVRNSKRGAAGSLMNVLNYPGMSHCVEITEGILADECAALLCDFYHMPRQVFNARKKAQSSINPGGSSGGSGGSETPGTSESATLENSGGSSGGSVKNTITKTLKLRIVRPYNSAEVEKIVADEKNNRERIALEKNKDKVKEACSKHLKVASYCTTQVERSACPFCKARKLDDKFYQELRGQFPDAVFWQEIGEIFRQLQKQAAEVYNQSLIELYYEIFIKGKGFANASSVEHYLSDVCYTRAAELFKNAAIASGLRGKVKSNFRLKELKNMKSGLPTTKSDNFPIPLVKQKGGQYTGFEISSHNDDFIIKIPFGRWQVKKEINKYRPWEKFDFEQVRKSPKPISLLLSTQRRKRNKGWSKDEGTEAEIRRVMNGDYQTSYIEVKRGSKIGEKSAWMLNLSIDVPKIDKGVDPSIIGGIDVGVKSPLVCAINNAFSRYSISDNDLFHFNKKMFARRRILLKKTRHKRAGHGAKNKLKPISILTEKSERFRKKLIERWACEIADFFIKNKVGTVQMENLESMKRREDSYFNIRLRGFWPYAKMQNKIEFKLKQYGIEIRKVAPNNTSKTCSKCGHLNNYFNFEYRKKNKFPHFKCEKCNFKENADYNAALNISNPKLKSTKEEH

SEQ ID NO: 2219 - protein, 726 aa, synthetic construct
SEVEFSHEYWMRHALTLAKRARDEREVPVGAILVLNNRVIGEGWNRTTSLHDPTAHAEIMALRQGGLVMQNHRLVDATLYVTFEPCVMCAGAMIHSRIGRVVFGVRNSKRGAAGSLTNVLNYPGMNHRVEITEGILVDECATLLCDFYRMPRQVFNAQKKAQSTINSGGSSGGSSGSETPGTSESPTPESSGGSPGGSAKNTITKTLKLRIVRPYNSTEVEKIVADEKNNREKIALEKNKDKVKEACSKHLKVAAYCTTQVERNACLFCKARKLDDKFYQKLRGQFPDAVFWQELGEIFRQLQKQAAEIYNQSLVELYYEIFIKGKGFANASSVEHYLSDVCYTRAAELFKNAAIASGLRGKVKSNFRLKELKNMKSGLPTTKSDNFPIPLVKQKGGQCTGFEISSHNDDLIVKIPFGRWQVKKEIDRYRPWEKFDFEQVRKSPKPISLLLSTQRRKRNKGWSKDEGTEAEIRKVMNGDYQTSYIEVKRGSKIGEKNAWMLNLSIDVPKIDKGVDPNIIGGIDVGVKSPLVCAINNAFSRYSISDNDLFRFNKKMFARRRILLKKNRHKRAGHGAKNKLKPISILTGKSERFRKKLIERWACEIADFFIKNKVGTVQMENLESMKRKEDSYFNIRLRGFWPYAEMQNKIEFKLKQYGIEIRKVAPNNTSKTCSRCGHLNNYFNFEYRKKSKFPHFKCEKCNFKENADYNAALNISNPKLKSTKEEP

SEQ ID NO: 2220 - protein, 726 aa, synthetic construct
SEVEFSHEYWMRHALTLAKRARNEREVPVGAILVLNNRVIGEGWNRAIGLHDPTAHAEIMALRQGGLVMQNYRLIDATLYVTFEPCVMCAGAMIHSRIGRVVFGVRNNKHGAAGSLVNVLNYPGMNHRVEITEGILADECAALLCDFYRMPRRVFNARKKAQSSTNPGGSSGGSSGSETPGTSESATPESSGGSSGGSAKNTITKTLKLRIVRPYNSAEVEKIVADEKNNREKIALEKNKDKVKEACSEHLKVAAYCTTQVERSACLFCKARKLDDKFYQKLRGQFPDAVFWQELGGIFRQLQKQAAEIYNQSLIELYYEIFIKGKGIASASRVGHYLSDVCYTRAAELFKNAAIASGLRNKIKSNFRLKELRNMKSGLPTTKSDNFPIPLVRQKGGQYTGFEISNHNGDFIIKIPFGRWQVKKEISKHRPWEKFDFEQVRKSPKPISLLLSTQRRKRNKGWSKDEGTEAEIRKVMNGDYQTSYIEVKRGSKIGEKSAWMLSLSIDVPKIDKGVDPSTIGGIDVGVKSPLVCAINNAFCRYSISDNDLFHFNKKMFARRRILLKKNRHKRAGHGAKNKLKPVSILTEKSKRFRKKLIERWACEIADFFIKNKVGTVQMENLESMKRKEDSYFNIRLRGFWPYAEMQNKIEFKLKQYGIEIRKVAPNNTSKTCSKCGHLNNYFNFEYRKKNKFPHFKCEKCNFMENADYNAALNISNPKLKSTKEEP

SEQ ID NO: 2221 - protein, 726 aa, synthetic construct; identical to SEQ ID NO: 684

SEQ ID NO: 2222 - protein, 726 aa, synthetic construct; identical to SEQ ID NO: 684

SEQ ID NO: 2223 - protein, 726 aa, synthetic construct
SEVEFSHEYWMRHALTLAKRARDEREVPVGAVLVLNNRVIGEGWNRAIGLHDPTAHAEIMALRQGGLVMQNYRLTDATLYVTFEPCVMCAGAMIHSRIGRVVFGVRNSKRGAAGSLMNVLNYPGMNHCVEITEGILMDECAALLCDFYRMPRQVLNAQKKAQSSISSGGPSGGSSGSEAPGTSESATPKSSGGSSGGSAKNTITKALKLRIVRPYNSAEVEKIVADEKNNRERIALEKNKDKVREACSEHLKVAAYCTTQVERSACLFCKARKLDDKFYQKLRGQFPDAVFWQEIGEIFRQLQKQAAEIYNQSLIELYYEIFIKGKGFANASSVEHYLSDVCYTRAAELFKNAAIASGLRGKVKSNFRLKELKNMKSGLPTTKSDNFPIPLVKQKGGQYTGFEISSHNDDFIIKIPFGRWQVKKEIDKYRPWEKFDFEQVRKSPKPISLLLSTQRRKRNKGWSKDESTEAEIRKVMNGDYQTSYIEVKRGRKIGEKSAWMLNLSIDVPKIDKGVDPSTIGGIDVGVKSPLVCAINSAFSRYSIGDNDLFHYNKKMFARRRILLKKNRHKRAGHGAKNKLKPISILTEKSERFRKKLIERWACEIADFFIKNKVGTVQMENLESMKRREDSYFNIRLRGFWPYAKMLNKIEIKLKQYGIKIRKVAPNNTSKTCSKCGHLNNYFNFEYRKKNKFPHFKCEKCNFKENADYNAALNISNPKLKSTKGEP

SEQ ID NO: 2224 - protein, 726 aa, synthetic construct
SEVEFSHEYWMRHALTLAKRARDEREVPVGAVLVLNNRVIGEGWNRAIGLHDPTAHAEIMALRQGGLVMQNYRLVDATLYVTFEPCVLCAGAMVHSRIGRVVFGVRNSKRGAAGSLMNVLNYPGMNHRVEITEGILADECAALLCDFYRMPRQVFNARKKARSNINSSGSSGGSSGSETPGTSESATPESSGGSSGGSAKNTITKTLKLRIVRPYNSAEVEKIVADEKDNREKIALEKNKDKVKEACSKHLKVASYCTTQVERNACPFCKARKLDDKFYQKLRGQFPDAVFWQELGEILRQLQKQAAEIYNQSLIELYYEIFIKGRGFANTSSVEHYLSDVCYTRAAELFKNAAIASGLRGKVKSNFRLKELKNMKSGLPTTKSDNFPIPLVKQKGGQYTGFEISNHDGDFIIRIPFGRWRVKKEINKHRPWEKFDFEQVRKSPKPISLLLSTQRRKRNKGWSKDEGTEAEIRKVMNGDYQTSYIEVKRGSKIGEKSAWMLNLSIDVPKIDKGVDPGIIGGIDVGVKSPLVCAINNALSRYSISDNDLFHFNKKMFARRRILLRKNRHKRAGHGAKNKLKPITMMTEKSKRFRKKLIERWACEIADFFIKNKVGTVQMEDLESMKRKEDSYFNIRLRGFWPYAEMQNKIEFKLKQYGIVVRKVAPNNTSKTCSKCGHLNNYFNFEYRKKNKFPHFKCEKCNFKENADYNAALNISNPQLKSTKGEP

SEQ ID NO: 2225 - protein, 726 aa, synthetic construct
SEVEFSHEYWMRHALTLAKRARDEREVPVGAVLVLNNRVIGEGWNRAIGLHDPTAHAEIMALRQGGLAMQNYRLVDATLYVTFEPCVLCAGAMVHSRIGRVVFGVRNSKRGAAGSLMNVLDYPGMDHRVEITEGILADECAALLCDFYRMPHQVFNAQKKAQSSINSGGSSGGSSGSVTPGTSESATPESSGGSSGGSAKNTITKTLKLRIVRPYNSAEVEKIVADEKNNREKIALEKNKDKVKEACSKHLKVAAYCTTQVERNACLFCKARRLDDKFYQKLRGQFPDAVFWQEIGEIFRQLQKQAAEVYNQSLVELYYEILIKGKGIANASSVEHYLSDVCYTRAAELFKNAAIASGLRNKIKSNFRLKELRNMKSGLPTTKSDNFPIPLVRQKGGQYTGFEISNHDGDFIIKIPFGRWQAKKEINKHRPWEKFDFEQVRRSPKPISLLLSTQRRKRNKGWSKDEGTEAEIRKVMNGDYQTSYIEVKRGSKIGEKSAWMLNLSIDVPKIDKGVDPSIIGGIDVGVKSPLVCAINNAFSRYSISDNDLFRFNKKMFARRRILLKKNRHQRAGHGAKNKLKPITILTEKSGRFRKKLIERWACEIADFFIKNKVGTVQMENLESMKRKEDSYFNIRLRGFWPYAEMQNKIEFKLKQYGIKIRKVAPNNTSKTCSKCGHLNNYFSFEYRRKNKFPHFKCEKCNFKEDADYNAALNISNPKLKSTKEEP

SEQ ID NO: 2226 - protein, 726 aa, synthetic construct; identical to SEQ ID NO: 684

SEQ ID NO: 2227 - protein, 726 aa, synthetic construct
SEVEFSHEYWMRHALTLAKRARDEREVPVGAILVLNNRVIGEGWNRAIGLHDPTAHAEIMALRQGGLVMQNYRLIDATLYVTFEPCVMCAGAMIHSRIGRVVFGARNSKHGAAGSLVNVLNHPGMNHRVEITEGILADECAALLCDFYRMPRQVFNARKKAQSSIYPGGSSGGSSGSETPGTSESATPESSGGSSGGSAKNTITKTLKLRIVRPYNSAEVEKIVADEKNNREKIALEKNRDKVKEACSKHLKVAAYCTTQVERNACLFCKARKLDDKFYQKLRGQFPDAVFWQEIGEIFRQLQKQAAEIYNQSLIELYYEIFIKGKGFANASSVEHYLSDVCYTRAAELFKNAAIASGLRGKVKSNFRLKELKNMKSGLPTTKSDNFPIPLVKQKGGQYTGFEISNRNSDFIIKIPFGRWQVKKEINKYRPWEKFDFEQVRKSPKPISLLLSTQRRKRNKGWSKDGGTEAEIRKVMNGDYQTSYIEVKRGSKTGEKSAWMLNLSIDVPKIDKGVDPSIIGGIDVGVKSPLVCAINNAFSRYSISDNDLFRFNKKMFARRRILLGKNRHKRAGHGVKNKLKPITILTEKSGRFRKKLIERWACEIADFFIKNKVGTVQMENLESMKRKEDSYFNIRLRGFWPYAEMQNRIEFKLKQYGIEIRKVAPNNTSKTCSKCGHLNNYFNFEYRKKNKFPHFKCEKCSFKENADYNAALNISSPKLKSTREEP

SEQ ID NO: 2228 - protein, 726 aa, synthetic construct
SEVEFSHEYWMRHALTLAKRARDEREVPVGAILVLNNRVIGEGWNRAIGLHDPTAHAEIMALRQGGLVMQNYRLIDATLYVTFEPCVMCAGAMIHSRIGRVVFGVRNSKRGAAGSLTNVLNYPGMNHRVEITEGILVDECAALLCDFYRMPRQVFNAQKKAQSTFNSGGSSGGSSGSETPGTSESPTPGSSGGSPGGSAKNTITKTLKLRIVRPYNSAEVEKIVADEKDNRERIALEKNKDKVKEACSKHLKVAAYCTTQVERNACLFCKARELDDKFYQKLRGQFPDAVFWQEIGEIFRQLQKQAAEIYNQSLIELYYEIFIKGKGFANASSVEHYLSDVCYTRAAELFKNAAIASGLRGKVKSNFRLKELKNMKSGLPTTKSDNFPIPLVKQKGGQYTGFEISSHNDDFIIKIPFGRWQVKKEIDKYRPWEKFDFEQVRKSPKPISLLLSTQRRKRNRGWSKDESTEAEIKKVMNGDYQTSYIEVKRGSKVGEKSAWMLNLSIDVPKIDKGVDPSIIGGIDVGVKSPLVCAINNAFSRYSISDNDLYRFNKKMFARRRILLKKSKHKRAGHGAKNKLKPITILTEKSGRFRKKLIERWACEIADFFIKNKVGTVQMENLESMKRKEDSYFNIRLRGLWPYAEMQNKIEFKLRQYGIEIRKVAPNNTSKTCSKCGHLNNYFNFEYRKKNKFPHFKCEKCNFKENADYNAALNISNPRLKSTKEEP

SEQ ID NO: 2229 - protein, 726 aa, synthetic construct; identical to SEQ ID NO: 2100

SEQ ID NO: 2230 - protein, 726 aa, synthetic construct
SEVEFSHEYWMRRALTLAKRARDEREVPVGAVLVLNNRVIGVGWNRAIGLHDPTAHAEIMALRQGGLVMRNYRLTDATLYVTFEPCVMCAGAMIHSRIGRVVFGVRNSKRGAAGSLMNVLNYPGMNHCVEITEGILVDECAALLCDFYRMPRQVLNAQKKAQSSISPGGSSGGSSGSETPGASESVTPKSSGGSSGGSAKNTITKTLKLRIVRPYNSAEVEKIVADEKNNREKIALEKNKGKVKEACSKHLEVAAYCTTQVERNACLFCKARKLDDKFYQKLRGQFPDAVFWQEIGEIFRQLQKQAAEIYNQSLIELYYEIFIKGKGITNASRVEHYLSDVCYTRAAELFKNAAIASGLRSKVRSNFRLKELRNMKSGLPTTKSDNFPIPLVKQKGGQHTGFEISSHNSDFIIKIPFGRWQVKKEIDKYRPWEKFDFEQVRKSPKPISLLLSTRRRKRNKGWSKDEGTEAEIRKVMNADYQTSYIEVKRGSKIGEKSAWMLNLSIDVPKIDKGVDPSIIGGIDVGVKSPLVCAINNAFSRYSISDNDLFRFNKKVFARRRILLKKNRHKRAGHGTKNKLKPITILTEKSGRFRKKLIERWACEIADFFIKNKVGTVQMENLESMKRKEDSYFNIRLRGFWPYAEMQNKIEFKLKQYGIEIRRVAPNNTSRTCSKCGHLNNYFNFEYRRKYKFPHFKCEKCNFKEDADYNAALNISNPKLKSTKEEP

SEQ ID NO: 2231 - protein, 726 aa, synthetic construct
SEVEFSHEYWMRHALTLAKRARDGREVPVGAVLVLNNRVIGEGWNRAIGLHDPTAHAEIMALRQGGLVTQNYRLIDATLYVTFEPCVMCAGAMVHSRIGRVVFGVRNSKRGAAGSLMNVLDYPGMGHRVEITEGILADECAALLCDFYCMPRQVFSAQKRAQSSINPGGSSGGSSGSETPGTSESPTPESSGGSSGGSAKNTITKTLKLRIVRPYNSAEVEKIVAEEKNNREKIALEKNKDKVKEACSKHLKVAAYCTTQVERNACLFCKARKLDDKFYQKLRGQFPDAVFWQEIGEIFRQLQKQAAEIYNQSLIELYYKIFIKGKGLANASNVEHYLSDVCYTRAAELFKNAAIASGLRGKVKSNFKLKELKSMKSGLPSTKSDNFPIPLVKQKGGQYTGFEISSHNDDFIIKIPFGRWQVKKEIDKYRPWEKFDFEQVRKSPKPISLLLSTQRRKRNKGWSKDEGTEAEIRKVMNGDYQTSYIEVKRGSKTGEKSAWMLNLSIDVPKIDKGVDPSIIGGIDVGVKSPLVCAINNALSRYSISDNDLFHFNKKVFARRRILLKKNGHKRAGHGARNKLKPITILTEKSKRFRKKLIERWACEIADFFIKNKVGTVQMENLESMKRKEDSYFNIRLRGFWPYAEMQDKIEFKLKQYGIEIRKVAPNNTSKTCSKCGHLNNYFNFEYRKKNKFPHFKCEKCSFKENADYNAALNISNPRLKSTKEEP

SEQ ID NO: 2232 - protein, 726 aa, synthetic construct; identical to SEQ ID NO: 684

SEQ ID NO: 2233 - protein, 726 aa, synthetic construct
SEVEFSHEYWMHHALTLAKRARDEREVPVGAVLVLNNRVIGVGWNRAIGLHDPTAHAEIMALRQGGLVMRNYRLTDATLYVTFEPCVMCAGAMIHSRIGRVVFGVRNSKRGAAGSLMNVLNYPGMNHCVEITEGILVDECAALLCDFYRMPRQVLNAQKKAQSSISPGGSSGGSSGSETPGACESVTPKSSGGSSGGSAKNTITKTLKLRIVRPHNSAEVEKIVADEKNNREKIALEKNKGKVKEACSKHLEVAAYCTTQVERNACLFCKARKLDDKFYQKLRGQFPGAVFWQELGEILRQLQKQAAEIYNQSLIELYYEIFIKGRGFANAGSVEHYLSDVCYTRAAELFKNAAIASGLRSKIKSNFRLKELKSMKSGLPTTKSDNFPIPLVKQKGGQYAGFEISNHNGDFIIKIPFGRWQVKKEVDRYRPWEKFDFEQVRKSPKSISLLLSTQRRKRNKGWSKDEGTEAEIRKVMNGDYQTSYIEVKRGSKIGEKSAWMLSLSIDVPKIDKGVDPSIIGGIDVGVKSPLVCAINNAFSRYSISDNDLFRFNKKMFARRRILLGKNRHKRAGHGVKNKLKPITILTEKSGRFRKKLIERWACEIADFFVKNKVGTVQMENLESMKRKEDSYFNIRLRGFWPYAEMQNKIEFKLKQYGIKVRKVAPNNTSKTCSKCGHLNNYFSFEYRKKNKLPHFKCEKCNFKENADYNAALNISNPKLKSTKEEP

SEQ ID NO: 2234 - protein, 726 aa, synthetic construct
SEVEFSHEYWMRHALTLAKRARDEREVPVGAVLVLNNRVIGEGWNRTIGLHDPTAHAEIMALRQGGLVMQNYRLTDATLYVTFEPCVMCAGAMIHGRIGRVVFGVRNSKRGAAGSLMNVLNCPGMNHCVEITEGILVDECAALLCDFYRMPRQVLNAQKKAQSSINSGGSSGGSSGSETPGTSESATPESSGGSSGGSAKNTITKTLTLRIVRPYNSAEVEKIVADEKNNREKIALEKNKDKVKEACSEHLKVATYCTTQVERNACPFCKARKLDDKFYQKLRGQFPDAVFWQELGEIFRQLRKQAAEIYNQSLIELYYEIFIKGKGIANASSVEHYLSDVCYTRAAELFKNAAIASGLRGKVKSNFRLKELRNMKSGLPTTKSDNFPIPLVRQKGGQYTGFEISSRNDDFIIKIPFGRWQVKKEIDKYRPWEKFDFEQVRKSPKPISLLLSTQRRKRNKGWSKDEGTEAEIKRVMNGDYQTSYIEVKRGSKIGEKSAWMLNLSIDVPKVDKGVDPSIIGGIDVGVKSPLVCAINNAFSRYSISDNDLFHFNKKMFARRRILLKKNRHRRAGHGAKNKLKPITILTEKSVRFRKKLIERWACEIADFFIKNKVGTVQMENLESMKRKEDSYFNIRLRGFWPYAEMQNKIEFKLKQYGIKIRKVAPNNTSRTCSKCGHLNNYFSFEYRKKNKFPHFKCEKCNFKENADYNAALNISNPKLKSTKGEP

SEQ ID NO: 2235 - protein, 726 aa, synthetic construct
SEVEFSHEYWMRHALTLAKRARDEREVPVGAVLVLNNRVIGAGWNRTTGLHDPTAHAEIMALRQGGLVMQNHRLVDATLYVTFEPCVMCAGAMIHSRIGRVVFGIRNSKRGAAGSLTNVLNYPGMSHRVEITEGILADECAALLCDFYRMPRQVFNAQKKAQSNINPGSSSGGSSGSETPGTSESATPGSSGGSTGGSAKNTITKTLKLRIVRPYNSAEVEKIVADEKNNREKIALEKNKGKVKEACSKHLEVAAYCTTQVERNACLFCKARKLDDKFYQKLRGQFPDAVFWQELGEIFRQLQKQAAEIYNQSLVELYYEILIKGKGIANASSVEHYLSDVCYTRAAELFKNAAIASGLRNKIKSNFRLKELRNMKSGLPTTKSDNFPIPLVRQKGGQYTGFEISNHDGDFIIKIPFGRWQVKKEINKHRPWEKFDFEQVRKSPKPISLLLSTQRRKRNKGWSKDEGTEAEIRKVMNGDYQTSYIEVKRGSKIGEKSAWMLNLSIDVPKIDKGVDPSIIGGIDVGVKSPLVCAINNALSRYSISDNDLFHFNKKMFARRRILLRKNRHKRAGHGAKNKLKPITVLTEKSERFRKKLIERWACEIADFFIKNKVGTVQMENLESMKRREDSYFNIRLRGFWPYAEMQSKIEFKLKQYGIKIRKVAPNNTSKTCSKCGHLNNYFNFEFRKKNKFPHFKCEKCNFKEDADYNAALNISNPKLKGTKEEP

SEQ ID NO: 2236 - protein, 726 aa, synthetic construct; identical to SEQ ID NO: 684

SEQ ID NO: 2237 - protein, 726 aa, synthetic construct
SEVEFSHEYWMRHALSLAKRARDEREVPVGAVLVLNNRIIGEGWNRAIGLHDPTAHAEIMALRQGGLVMQNYRLVEATLYVTFEPCIMCAGAMIHGRIGRVVFGVRNSKRGAAGSLMNVLNYPGMNHCVEITEGILVDECAALLCDFYRMPRQVLNAQKKAQSSINSGGSSGGSSGSVTPGTSESATPESSGGSFGGSAKNTITKTLQLRIVRPYNSAEVEKIVADEKNSREKIALEKNKDKVKEACGKHLKVASYCTTQVERNACLFCKARKLDDKFYQKLRGQFPDAVFWQELGEIFRQLQKQAAEIYNQSLIELYYEIFIKGKGLANASSVEHYLSDVCYARAAELFKNAAIASGLRGKVKSNFKLKELKSMKSGLPSTKSDNFPIPLVKQKGGQYTGFEISSHNDDLIIKIPFGRWQVKKEIDKYRPWEKFDFEQVRKSPKPISLLLSTQRRKRNKGWSKDEGTEAEIRKVMNGGYQTSYIEVKRGSKIGEKSAWMLSLSIDMPKIDKGVDPSIIGGIDVGVKSPLVCAINNTLSRYSISDNDLFHFNKKMFARRRILLRKNRHKRAGHGAKNKLKPITIMTEKSKRFRKKLIERWACEIADFFIKNKVGTVQMENLESMKRKEDSYFNIRLRGFWPYAEMQNKIEFKLKQYGIVVRKVAPNNTSKTCSKCGHLNNYFNFEYRKKNKFPHFKCEKCNFKEDADYNAALNISNPKLKSTKGEP

SEQ ID NO: 2238 - protein, 726 aa, synthetic construct; identical to SEQ ID NO: 684

SEQ ID NO: 2239 - protein, 726 aa, synthetic construct
SEVEFSHEYWMRHALTLAKRARGEREVPVGAILVLNNRVIGEGWNRAIGLHDPTAHAEIMALRQGGLVMQNYRLTDATLYVTFEPCVMCAGAMIHSRIGRVVFGVRNNKHGAAGSLVNVLNYPGMNHRVEITEGILADECAALLCDFYRMPRQVFNARKKAQSSINPGGSSGGSSGSETPGTRESATPKNSGGSSGGSAKNTITKALKLRIVRPYNSAEVEKIVADEKNNRERIALEKNKDKVKEACSKHLKVAAYCTTQVERNACLFCKARKLDDKFYQKLRGQFPDAVFWQEIGEIFRQLQKQAAEIYNQSLIELYYEIFIKGKGFANASSVEHYLSDVCYTRAAELFKNAAIASGLRGKVKSNFRLKELKNMRSGLPTTKSDNFPIPLVKQKGGQYAGFEISSHNDDFIIKIPFGRWQVKKEIDKYRPWEKFDFEQVRKSPKPISLLLSTRRRKKNKGWSKDEGTEAEIRKVMNGDYQTSYIEVKRGSKIGEKSAWMLNLSIDVPKIDKGVDPSIIGGIDVGVKSPLVCAINNAFGRYSISDNDLFHFNKKMFARRRILLKKNRHKRAGHGAKNKLKPISILTGKSERFRKKLIERWACEIADFFIKNKVGTVQMENLESMKRKEDSYFNIRLRGFWPYAEMQNKIEFKLKQYGIEIRKVAPNNTSKTCSKCGHLNNYFNFEYRKKNKYPHFKCEKCNFKENADYNAALNISNPKLKSTREEP

SEQ ID NO: 2240 - protein, 726 aa, synthetic construct
SEVEFSHEYWMRHALTLAKRARDEREVPVGAILVLNNRVIGEGWNRAIGLNDPTAHAEIMALRQGGLVMQNYRLIDATLYVTFEPCVMCAGAMIHSRIGRVVFGVRNNKHGAAGSLVNVLNYPGMNHRVEITEGILADECAALLCDFYRMPRQVFNARKKAQSSINPGGSSGGSGGSETPGTSESPTPESSGGSFGGSAKNTITKTLQLRIVRPYNDAEVEKIVADEKNSREKIALEKNKDKVKEACGKHLKVASYCTTQVERNACLFCKARKLDDKFYQKLRGQFPDAVFWQELGEIFRQLQKQAAEIYNQSLIELYYEIFIKGKGLANASSVEHYLSDVCYTRAAELFKNAAIASGLRGKVKSNFKLKELKSMKSGLPSTKSDNFPIPLVKQKGGQYTGFEISSHNDDLIIKIPFGRWQVKKEVDKYRPWEKFDFEQVRKSPKPITLLLSTQRRKRSKGWSKDEGTEAEIRKVMNGDYQTSYIEVKRGSKIGEKCAWMLNLSIDVPKIDKGVDPSIIGGIDVGVKSPLVCAINNAFSRYSISDNDLFRFNKKMFARRRILLKRNRHKRAGHGAKNKLKPITVLTEKSERFRKKLIERWACEIANFFIKNKVGTVQMENLESMKRREDSYFNIRLRGFWPYAEMQNKIEFKLKQYGIKIRKVAPNNTSKTCSQCGHLNNYFNFEYRKKNKFPHFKCEKCNFREDADYNAALNISNPKLKSTKEEP

SEQ ID NO: 2241 - protein, 726 aa, synthetic construct
SEVEFSHEYWMRHALTLAKRARDEREVPVGAVLVLNNRVIGEGWNRAVGLHDPTAHAEIMALRQGGLVMQNYRLIDATLYVTFEPCVMCAGAMIHSRIGRVVFGVRNSKRGAAGSLMNVLNYPGMNHCVEITEGILVDECAALLCDFYRMPRQVLNAQKKAQSSISSGGSSGGSSCSETPGASESVTPKSSGGGSAGSTKNTITKTLKLRIVRPYNSAEVEKIVADEKNSREKIALEKNKDKVKEACSKHLKVASYCTTQVERNACPFCKARKLDDKFYQKLRGQFPDAVFWQELGEILRQLQKQAAEIYNQSLVELYYEVFIKGRGFANASSVEHYLSDVCYTRAAELFKNAAIASGLRGKVKSNFRPKELKNMKSGLPTTKSDNFPIPLVKQKGGQYTGFEISSHNDDFIIKIPFGRWQAKKEIDKYRPWEKFDFEQVRKSPKPISLLLSTQRRKRNKGWSKDEGTEAEIRKVMNGDYQTSYIEVKRGSKTGEKSAWMLNLSIDVPKVDKGVDPSIIGGIDVGVKSPLVCAINNAFSRYSISDNDLFRFNKKMFARRRILLKKNRHKRAGHGAKNKLKPISILTGKSERFRRKLIERWACEIADFFIKNKVGTVQMENLESMKRKEDSYFNIRLRGFWPYAEMQDKIEFKLKQYGIVVRKVAPNNTSKTCSKCGHLNNYFNFEYRKKNKFPHFKCEKCNFKEDADYNAALNISNPKLKSTKGEP

SEQ ID NO: 2242 - protein, 726 aa, synthetic construct
SEVEFSHEYWMRHALTLAERARDEREVPVGAVLVLNNRVIGEGWNRAIGLHDPTAHAEIMALRQGGLVMQNYRLTDATLYVTFEPCVMCAGAMIHSRIGRVVFGVRNSKHGAAGSLVNVLNYPGMNHRVEITEGILADECTALLCDFYRMPRQVFNARKKAQSSISPDGSSGGSSGSETPGTSESATPESSGGSSGGSAKNTITKTLKLRIVRPYNSAEVEKIVADEKNNRERIALEKNKDKVKEACSKHLKVAAYCTTQVERNACLFCKARRLDDKFYQELRGRFPDAVFWQEIGEIFRQLQKQAAEIYNQSLIELYYEIFIKGKGFANASSVEHYLSDVCYTRAAELFKNAAIASGLRGKVKGNFKLKELKSMKSGLPSTKSDNFPIPLVKQRGGQYTGFEISSHNDDFIIKIPFGRWQAKKEIDKYRPWEKFDFEQVRKSPKPISLLLSTQRRKRNKGWSKDEGTEAEIRKVMNGDYQTSYIEVKRGSKIGEKSAWMLNLSIDVPKIDKGVDPSIVGGIDVGVKSPLVCAINNAFSRYSISDNDLFHFNKKMFARRRILLKKNRHKRAGHGAKNKLKPITIMTEKSKRFRKKLIERWACEIADFFIKNKVGTVQMENLESMRRKEDSYFNIRLRGFWPYAEMQNKIEFKLKQYGIEIRRVAPNNTSRTCSKCGHLNNYFNFEFRKKNKFPHFKCEKCNFKEDADYNAALNISNPKLKSTKEEP

SEQ ID NO: 2243 - protein, 726 aa, synthetic construct
SEVEFSHEYWMRHALTLARRARDEREVPVGAILVLNNRVVGEGWNRAIGLHDPTAHAEIMALRQGGLVMQNYRLTDATLYVTFEPCVMCAGAMIHSRIGRVVFGVRNSKHGAAGSLVNVLNYPGMNHRVEITEGILADECAALLCDFYRMPRQVFNARKKAQSSINPGGSSGGSSGSETPGTSEGATLENSGGSSGSSAKNTITKTLQLRIVRPYNSAEVEKIVADEKNNREKIALEKNKDKVKEACSKHLKVASYCTTQVERNACPFCKARKLDDKFYQKLRGQFPDAVFWQETGEIFRQLQRQAAEIYNQSLIELYYEIFIKGKGFANASSVEHYLSDVCYTRAAELFKNAAIASGLRGKVKGNFRLKELKNMKSGLPTTKSDNFPIPLVKQKGGQYTGFEISSHNDDFIIKIPFGRWQAKKEIDKYRPWEKFDFEQVRKSPKPISLLLSTQRRKRNKGWSKDEGTEAEIRRVMNGDYQTSYIEVKRGSKIGEKSAWMLNLSIDVPKIDKGVDPSIIGGIDVGVKSPLVCAINNAFSRYSISDNDLFHFNKKMFARRRILLKRNRRRRAGHGAKNKLKPITILTEKSVRFRKKLIERWACEIADFFIKNKVGTVQMENLESMKRKEDSYFNIRLRGFWPYAEMQNKIEFKLKQYGIEIRRVAPNNTSRTCSKCGHLNNYFNFEYRRKYKFPHFKCEKCNFKEDADYNAALNISNPKLKSTKEEP

SEQ ID NO: 2244 - protein, 726 aa, synthetic construct
SEVEFSHEYWMRHALTLAKRARDEREVPVGAVLVLNNRVIGEGWNRAIGLHDPTAHAEIMALRQGGLAMQNYRLVDATLYVTFEPCVLCAGAMVHSRIGRVVFGVRNSKRGAAGSLMNVLNHPGMNHRVEITGGILADECAALLCDFYRMPRQVFNARKKAQSSINPGGSSGGSSGSETPGTSESATLENSGGSSGGSAKNTITKTLKLRIVRPYNSAEVERIVADEKNNREKIALEKNKDKVKEACSKHLKVAAYCTTQVERNACLFCKARRLDDKFYQKLRGQFPDAVFWQEIGEIFRQLQKQAAETYNQSLIELYYEIFIKGKGIANASNVEHYLSDVCYTRAAELFKNAAIASGLRNKIKSNFRLKELRNMKSGLPTTKSDNFPIPLVKQKGGQYTGFEISNHNGDFIIKIPFGRWQAKKEIDKYRPWEKFDFEQVRKSPRPISLLLSTQRRKRNKGWSKDEGTEAEIRKVMNGDYQTSYIEVKRGSKIGEKSAWMLNLSIDVPKIDKGVDPSIIGGIDVGVKSPLVCAINNAFCRYSISDNDLFHFNKKMFARRRILLKKSRHKRAGHGAKNKLKPISILTEKSKRFRKKLIERWACEIADFFIKNKVGTVQMENLESMKRKEDSYFNIRLRGFWPYAEMQNKIEFKLKQYGIEIRKVAPNNTSKTCSKCGHLNNYFNFEYRKKNKFPHFKCEECNFKENADYNAALNISNPKLKSTKEEP

SEQ ID NO: 2245 - protein, 726 aa, synthetic construct
SEVEFSHEYWMRHALTLAKRARDEREVPVGAVLVLNNRVIGEGWNRAIGLHDPTAHAEVMALRQGGLVMQNYRLTDATLYVTFEPCVMCAGAMIHGRIGRVVFGVRNSKRGAAGSLMNVLNYPGMNHCVEITEGILVDECAALLCDFYRMPRQVLNAQKKAQSSISPGGSSGGSSGSETPGASGSVTPKSSGGGSAGSTKDTITKTLKLRIVRPYNSAEVEKIVADEKNSREKIALEKNKDKVKEACSEHLKVAAYCTTQVERNACLFCKARKLDDRFYQKLRGQFPDAVFWQEIGEIFRQLQKQAAEIYNQSLIELYYEIFIKGKGFANASSVEHYLSDVCYTRAAELFKNAAIASGLRGKVKSNFRLKELKNMKSGLPTTKSDNFPIPLVKQKGGQYTGFEISSRNDDFIIKIPFGRWQVKKEIDKYRPWEKFDFEQVRKSPKPISLLLSTQRRKRNKGWSKDEGTEAEIKKVMNGDYQTSYIEVKRGSKIGEKSAWMLNLSIDVPMIDKGVDPSIIGGIDVGVKSPLVCAINNAFSRYCISDNDLFHFNKKMFARRRILLKKNRHRRSGHGAKNKLKPITILTEKSGRFRKKLIERWACEIADFFIKNKVGTVQMEDLESMKRKEDSYFNIRLRGLWPYAEMQNKIEFKLKQYGIKIRKVAPNNTSKTCSKCGHLNNYFNFEYRKKNKFPHFKCEKCNFKENADYNAALNISNPKLKSTKEEP

SEQ ID NO: 2246 - protein, 726 aa, synthetic construct
SEVVFSHEYWMRHALTLAKRARDEREVPVGAVLVLNNRVIGEGWNRAIGLHDPTAHAEIMALRQGGLVMQNYRLIDATLYVTFEPCVMCAGAMVHSRIGRVVFGVRNSKRGAAGSLMNVLDYPGMGHCVEITEGILADECAALLCDFYCMPRQVFNAQKRAQSSINSGGSSGGSSGSETPGTSESATPESSGGGSSGSAKNTITKTLQLRIVRPYNSAEVEKIVADEKNNREKIALEKNKDKVKEACSKHLKVASYCTTRVERNACPFCKARKLDDKFYQKLRGQFPDAVFWQELGEIFRQLQKQAAEIYNQSLIELYYEIFIKGKGFANASSVEHYLSDVCYTRAAELFKNAAIASGLRGKVKSNFRLKELKNMKSGLPTTRSDNFPIPLVKQKGGQYTGFEISNHNSDFIIKIPFGRWQVKKEIDKYRPWEKFDFAQVRKSPKPISLLLSTQRRKRNRGWSKDESTEAEIRKVMNGDYQTSYIEVKRGSKIGEKSAWMLNLSIDVPKIDKGVDPSIIGGIDVGVKSPLVCAINNVLSRYSISDNDLFHFNKKMFARRRILLKKNGHKRAGHGAKNKLKPITIMTEKSKRFRKKLIERWACEIADFFIKNKVGTVQMENLESMKRKEDSYFNIRLRGFWPYAEMQNKIEFKLKQYGIVVRKVAPNNTSKTCSQCGHLNNYFNFEYRKKNKFPYFKCEKCNFKENADYNAALNISNPQLKSTKGEP

SEQ ID NO: 2247 - protein, 726 aa, synthetic construct
SEVEFSHEYWMRHALTLAKCARDEREVPVGAILVLNNRVIGEGWNRAIGLHDPTAHAEIMALRQGGLVMQNYRLIDATLYVTFEPCVMCAGAMIHSRIGRVVFGVRNNKHGAAGSLVNVLNYPGMNHRVEITEGILANECAALLCDFYRMPRQVFNARKKAQSSINPGGSSGGSSGSETPGTSESATPESSGGSSGGSAKNTITKTLKLRIVRPYNSAEVEKIVADEKNNREKIALEKNKDKVKEACSKHLKVAAYCTTQVERNACLFCKARRLDDKFYQKLRGQFPDAVFWQEIGEIFRQLQKQAAEIYNQSLVELYYEILIKGKGIANASSVEHYLSDVCYTRAAELFKNAAIASGLRNKIKSNFRLKELRNMKSGLPTTKSDNFPIPLVRQKGGRYTGFEISNHNGDFIIKIPFGRWQVKREINKHRPWEKFDFEQVRKSPKPISLLLSTQRRKRNKGWSKDEGTEAEIRKVMNGDYQTSYIEVKRGSKIGEKSAWMLNLSIDVPKIDKGVDPSIIGGIDVGVKSPLVCAINNALSRYSISDNDLFHFNKKMFARRRILLKKNRHKRAGHGAKNKLKPITILTEKSKRFRKKLIERWACEIADFFIKNKVGTVQMEDLESMKGKEDSYFNIRLRGFWPYAEMQSKIEFKLKQYGIKIRKVAPNNTSRTCSKCGHLNNYFSFEYRKKNKFPHFKCEKCNFKEDADYNAALNISNPKLKGTKEEP

SEQ ID NO: 2248 - protein, 726 aa, synthetic construct
SEVEFSHEYWMRHALTLAKRARDEREVPVGAILVLNNRVIGEGWNRAIGLQDPTAHAEIMALRQGGLVMQNYRLSDATLYVTFEPCVMCAGAMIHSRIGRVVFGVRNSKRGAAGSLMNVLNYPGMNHCVEITEGILVDECAALLCDFYRMPRQVLSAQKKAQSSVSSGGSSGGSSGSETPGASGSVTPKSSVGSSAGSTKNTITKTLKLRIVRPYNSAEVEKIVADEKNSREKIALERNKDKVKEACSKHLKVASYCTTQVERNACPFCKARKLDDKFYQKLRGQFPDAVFWQEIGEIFRQLQKQAAEIYNQSLVELYYEIFIKGKGIANASSVEHYLSDVCYTRAAELFKNAAIASGLRNKIKSNFRLKELRNMKSGLPTTKSDNFPIPLVRQKGGQYTGFEISNHNGDFIIKIPFGRWQVKKEICKHRPWEKFDFEQVRKSPKPISLLLSTQRRKKNRGWSKDEGTEAEIKKVMNGDYQTSYIEVKRGSKIGEKSAWMLNLSIDVPKIDKGVDPSIIGGIDVGVKSPLVCAISNAFSRYSISDNDLFHFNKKMFARRRILLKKSKHKRAGHGAKNKLKPITILTEKSRRFRKKLIERWACEIADFFIKNKVGTVQMENLESMKRKEDSYFNIRLRGFWPYAEMQNKIEFKLKQYGIEVRKVAPNNTSKTCSKCGHLNNYFNFEYRKRNKFPHFKCEKCNFKEDADYNAALNISNPKLKGTKEEP

SEQ ID NO: 2249 - protein, 725 aa, synthetic construct
SEVEFSHEYWMRHALTLAKRARDEREVPVGAVLVLNNRVIGEGWNRAIGLHDPTAHAEIMALRQGGLVMQNYRLTDATLYVTFEPCVMCAGAMIHSRIGRVVFGVRNSKRGAAGSLMNVLNYPGMNHCVEITEGILVDECAALLCDFYRMPRQVLNAQKKAQSSISPGGSSGGSSGSETPGAGESVTPKSSVGSSAGSTKNTITKTLKLRIVRPYNSAEVEKIVADEKNNREIALEKNKDKVKEACSKHLKVASYCTTQVERNACPFCKARRLDDKFYQKLRGQFPDAVFWQEIGEIFRQLQKQAAEIYNQSLVELYYEILIKGKGIANASSVEHYLSDVCYTRAAELFKNAAIASGLRNKIKSNFRLKELRNMKSGLPTTKSDNFPIPLVKQKGGQYTGFEISSHNDDFIIKIPFGRWQVKEEIGKYRPWEKFDFEQVRKNPKPISLLLSTQRRKRNKGWSKDEGTEAEIRKVMNGDYQTSYIEVKRGSKIGEKSAWMLNLSIDVPKIDKGVDPSIIGGIDVGVKSPLVCAINNAFSRYSISDNDLFRFNKKVFARRRILLKKNRHKRAGHGTKNKLKPITILTEKSGRFRKKLIERWACEIANFFIKNKVGTVQMENLESMKRRGDSYFNIRLRGFWPYAEMQNKIEFKLKQYGIKIRKVAPNNTSKTCSKCGHLNNYFNFEYRKKNKFPHFKCEKCDFREDADYNAALNISNPKLKSTKEEP

SEQ ID NO: 2250 - protein, 726 aa, synthetic construct
SEDEFSHEYWMRHALTLAKRARDGREVPVGAVLVLNNRVIGEGWNRAIGLHDPTAHAEIMALRQGGLVMQNYRLIDATLYVTFEPCVMCAGAMVHSRIGRVVFGVRNSKRGAAGSLMNVLDYPGMGHRVEITEGILADECAALLCDFYCMPRQVFNAQKRAQSSINSGGSSGGSSGSETPGTSESATPESSGGGSSGSAKNTITKTLQLRIVRPYNSAEVEKIVADEKNNREKIALEKNKDKVKEACSKHLKVASYCTTQVERNACPFCKARKLDDKFYQKLRGQFPDAVFWQELGEILRQLQKQAAEIYNQSLIELYYEIFIKGRGFANASSVEHYLSDVCYTRAAELFKNAAIASGLRGKVKSNFRLKELKNMKSGLPTTKSDNFPIPLVKQKGGQYTGFEISSYNDDLIIKIPFGRWQVKKEIDKYRPWEKFDFEQVRKSPKPISLLLSTQRRKRNKGWSKDEGTEAEIRKVMNGDYQTSYIEVKRGSKIGEKSAWMLNLSINVPKIDKGVDPSIIGGIDVGVKSPLVCAINNAFSRYSISDNDLFRFNKKMFARRRILLKKNRHKRAGHGAKNKLKPISILTERSERFRKKLIERWACEIADFFIKNKVGTVQMENLESMKRKEDSYFNIRLRGFWPYAEMQNKIEFKLKQYGIEIRKVAPNNTSKTCSKCGHLNNYFNFEYRKKNKFPHFKCEECNFKENADYNAALNISNPKLKSTKGEP

SEQ ID NO: 2251 - protein, 726 aa, synthetic construct
SEDEFSHEYWMRHALTLAKRARDGREVPVGAVLVLNNRVIGEGWNRAIGLHDPTAHAEIMALRQGGLVMQNYRLIDATLYVTFEPCVMCAGAMVHSRIGRVVFGVRNSKRGAAGSLMNVLDYPGMGHRVEITEGILVDECAALLCDFYRMPRQVFNARKKAQSSINPGGSSGGSGGSETPGTSESATPENSGGSSGSSAKNTITKTLKLRIVRPYNSAEVEKIVADEKNNREKIALEKNKDKVKEACSRHLKVAAYCTTQVERNACLFCKARKLDDKFYRKLRGQFPDAVFWQEIGEIFRQLQKQAAEIYNQSLIELYYEIFIKGKGIANASSVGHYLSDVCYARAAELFKNAAIASGLRSKIKSNFRLKELRNMRGGLPTTKSDNFPIPLVKQKGGQYTGFEISSHNDDFIIKIPFGRWQVKKEIDKYRPWEKLDFEQVRKSPKPISLLLSTQRRKRNKGWSKDEGTEAEIRKVMNGDYQTSYIEVKRGSKIGEKSAWMLNLSIDVPKIDKGVDPSIVGGIDVGVKSPLVCAIDNVLSRYSISDNDLFHFNKKMFARRRILLKKNRHRRAGHGAKNKLKPISILTEKSKRFRKKLIERWACEIADFFIKNKVGTVQMENLESMKRKEDSYFNIRLRGFWPYAEMQNKIEFKLKQYGIEIRKVAPNNTSKTCSKCGHLNNYFNFEYRKKNKFPHFKCEKCNFKENADYNAALNISNPMLKSTKEEP

SEQ ID NO: 2252 - protein, 726 aa, synthetic construct
SEVEFSHEYWMRHALSLAKRARDEREVPVGAVLVLNNRIIGEGWNRAIGLHDPTAHAEIMALRQGGLVMQNYRLTDATLYVTFEPCVMCAGAMVHSRIGRVVFGVRNSKRGAAGSLMNVLNYPGVNHCVEITEGILVDECAALLCDFYRMPRRVLNAQKKAQSSISSGGSSGGRSGSEMPGASESVTPKSSGGGFGGSAKNTITKTLQLRIVRPYNSAEVEKIVADEKNNREKIALEKNKDKVKEACSKHLKVASYCTTQVERNACLFCKARKLDDKFYQKLRGQFPDAVFWQELGEIFRQLQKQAAEIYNQSLIELYYEIFIKGKGLANASSVEHYLSDVCYTRAAELFKNAAIASGLRGKVKSNFKLKELKSMKSGLPSTKSDNFPIPLVKQRGGQYTGFEISSHNDDFIIKIPFGRWQAKKEIDKYRPWEKFDFEQVRKSPKPISLLLSTQRRKRNKGWSKDEGTEAEIKKVMNGDYQTSYIEVKRGSKIGEKSAWMLNLSIDVPRIDKGVDPSIIGGIDVGVKSPLVCAINNAFSRYSISDNDLFRFNKKMFARRRILLGKNRHKRAGHGVKNKLKPITILTEKSGRFRKKLIERWACEIADFFVKNKVGTVQMENLESMKRREDSYFNVRLRGFWPYAEMQNKIEFKLKQYGIEIRKVAPNNTSKTCSKCGHLNNYFNFEYRKKNKFPHFKCEKCNFKENADYNAALNISNPKLKSTKEEP

SEQ ID NO: 2253 - protein, 726 aa, synthetic construct
SEVEFSHEYWMRHALTLAKRARDEREVPVGAILVLNNRVIGEGWNRAIGLHDPTAHAEIMALRQGGLVTQNYRLIDATLYVTFEPCVMCAGAMIHSRIGRVVFGVRNNKHGAAGSLVNVLNYPGMNHRVEITEGILADECAALLCDFYRMPRQVFNARKKAQSSINPSGSSGGSSGSETPGTSESATPKSSGGSSAGSTKDTITKTLKLRIVRPYNSAEVEKVVADEKNNREKIAMEKNKDKVKEACSEHLKVAAYCTTQVERSACLFCKARKLDDKFYQKLRGQFPDAVFWQEIGEIFRQLQKQAAEIYNQSLIELYYEIFIKGKGITNASRVEHYLSDVCYTRAAELFKNAAIASGLRSKVRSNFRLKELKNMKSGLPTTKSDNFPIPLVKQKGGQYTGFEISSHNSDFIIKIPFGRWQVKEEIDKYRPWEKFDFEQVRKSPKPISLLLSTQRRKKNKGWSKDEGTEAEIRRVMNGDYQTSYIEVKRGSKIGEKSAWMLNLSIDVPKIDKGVDPSIIGGIDVGVKSPLVCAINNTFSRYSISDNDLFHYNKKMFARRRILLGKNRHKRAGHGTKNKLKPITILTEKSKRFRKKLIERWACEIADFFIKNKVGTVQMENLGSMKGKEDSYFNIRLRGFWPYAEMQNKIELKLRQYGIKIRKVAPNNTSKTCSKCGHLNDYFSFEYRKKNKFPHFKCEKCNFKEDADYNAALNISNPKLKSTREEP

SEQ ID NO: 2254 - protein, 726 aa, synthetic construct
SEVEFSHEYWMRHALTLAKRARDEREVPVGAILVLNNRVIGEGWNRAIGLHDPTAHAEIMALRQGGLEMQNYRLIDATLYVTFEPCVMCAGAMIHSRIGRVVFGVRNNKHGAAGSLVNVLNYPGMNHRVEITEGILADECAALLCDFYRMPRQVFNARKKAQSSINPGGSSGGSSGSETPGTSESATPESSGGSSGSSAKNTITKTLRLRIVRPYNSAEVEKIVADEKNNREKIALEKNKDKVKEACSKHLKVAAYCTTQVERNACLFCKARRLDDKFYQKLRGQFPDAVFWQEIGEIFRQLQKQAAEVYNQSLVELYYEILIKGKGIANASSVEHYLSDVCYTRAAELFKNAAIASGLRNKIKSNFRLKELRNMRSGLPTTKSDNFPIPLVRQKGGQYTGFEISNHDGDFIIKIPFGRWQVKEEINKHRPWEKFDFEQVRKSPKPISLLLSTQRRKRNKGWSKDEGTEAEIRKVMKGDYQTSYIEVKRGSKIGEKSAWMLNLSIDVPKIDKGVDPSIIGGIDVGVKSPLVCAINNALSRYSISDNDLFHFNKKMFARRRILLRKNRHKRAGHGAKNKLKPITMMTEKSKRFRKKLIERWACEIADFFIKNKVGTVQMENLESMKRKEDSYFNIRLRGFWPYAEMQNKIEYKLKQYGIEIRRVAPNNTSRTCSKCGHLNNYFNFEYRRKYKFPHFKCEKCNFKEDADYNAALNISNPKLKSTKEEP

SEQ ID NO: 2255 - protein, 726 aa, synthetic construct
SEVEFSHEYWMRHALTLAKRARDEREVPVGAILVLNNRVIGEGWNRAIGLHDPTAHAEIMALRQGGLVMQNYRLVDATLYVTFEPCVMCAGAMIHSRIGRVVFGVRNNKHGAAGSLVNVLNYPGMNHCVEITEGILVDECAALLCDFYRMPRQVLNAQKKAQSSISSGGSSGGSSGSVTPGASGSVTPKSSGGSSAGSTKDTITKTLKLRIVRPYNSAEVEKIVADEKNNREKIALEKNKDKVKEACSKHLKVASYCTTQVERNACPFCKARKLDDKFYQKLRGQFPDAVFWQELGEILRQLQKQAAGIYNQSLIELYYEIFIKGRGFANASSVEHYLSDVCYTRAAELFKNAAIASGLRGKVKSNFRLKELKNMKSGLPTTKSDNFPIPLVKQKGGQYTGFEINSHNGDFIIKIPFGRWQVKKEIDKYRPWEKFDFEQVRKGPKPISLLLSTRRRKRNKGWSKDEGTEAEIRKLMNGDYQTSYIEVKRGSRIGEKNAWMLNLSIDVPKVDKGVDPSIIGGIDVGVRSPLVCAINNAFSRYSVSDNDLFRFNKKMFARRRILLKKNRHKRAGHGAKNKLKPITILTEKSVRFRKKLIERWACEIADFFVKNKVGTVQMENLESMKRKEDSYFNIRLRGFWPYAEMQNKIEFKLKQYGIEIRKVAPNNTSKTCSKCGHLNNYFNFEYRKKNKFPHFKCEKCSFKENADYNAALNISNPKLKGTKEEP

SEQ ID NO: 2256 - protein, 726 aa, synthetic construct
SEVEFSHEYWMRHALTLAKRARDEREVPVGAVLVLNNRVIGEGWNRAIGLHDPTAHAEIMALRQGGLVMQNYRLSDATLYVTFEPCVMCAGAMIHSRIGRVVFGVRNSKRGAAGSLMNVLNYPGMNHCVEITEGILVDECAALLCDFYRMPRQVLSAQKKAQSSISSGGSSGGSSGGDTPGTSKSATPESSGGGSSGSAKNTITKTLQLRIVRPYNSAEVEKIVADEKNNREKIALEKNKDKVKEACSKHLKVASYCTTQVERNACPFCKARKLDDKFYQKLRGQFPDAVFWQELGEILRQLQKQAAEIYNQSLIELYYEIFVKGKGFANASSVEHYLSDVCYTRAAELFKNAAIASGLRGKVKSNFRLRELKSMRSGLPTTKSDNFPIPLVKQKGGQYTGFEISNHNSDFIIKIPFGRWQVKKEINKYRPWEKFDFEQVRKSPKPISLLLSTQRRKRNKGWSKDEGTEAEIRKVMNGDYQTSYIEVKRGSRIGEKSAWMLSLSIDVPKIDRGVDPSIIGGIDVGVKSPLVCAINNGLSRYSISDNDLFHFNKKMFARRRILLKKNRHRRAGHGARNKLKPITVLTEKSKRFRKKLIERWACEIANFFVKNKVGTVQMENLESMKRKEDSYFNIRLRGLWPYAEMQNKIEFKLKQYGIEIRKVAPNNTSKTCSKCGHLNNYFNFEYRKRNKFPHFKCEKCSFKENADYNAALNISNPKLKGTKEEP

SEQ ID NO: 2257 - protein, 726 aa, synthetic construct
SEVEFSHEYWMRHALTLAKRARDEREVPVGAILVLNNRVIGEGWNRAIGLHDPTAHAEIMALRQGGLVMQNYRLIDATLYVTFEPCVMCAGAMIHSRIGRVVYGVRNSKRGAAGSLMNVLDYPGMGHRVEITEGILADECAALLCDFYCMPRQVFNAQKRAQSSISSGGPSGGSSCSETPGASESVTPKSSGGSSAGSAKNTITKTLQLRIVRPYNSAEVEKIVADEKNNREKIALEKNKDKVREACSKHLKVASYCTTQVERNACPFCKARKLDDKFYQKLRGQFPDAVFWQELGEILRQLQKQAAEIYNQSLIELYYEIFIKGRGFANASSVEHYLSDVCYTRAAELFKNAAIASGLRGKVKSNFRLKELKNMKSGLPTTKSDNFPIPLVRQKGGQYTGFEISNHDGDFIIKIPFGRWQVKKEINKHRPWEKFDFEQVRRSPKPISLLLSTQRRKRNKGWSKDEGTEAEIRKVMNGDYQTSYIEVKRGSKIGEKSAWMLNLSIDVPKIDKGVDPSIIGGIDVGVKSPLVCAINNALSRYSISDNDLFHFNKKMFARRRILLRKNRHKRAGHGAKNKLKPITIMTEKSKRFRKKLIERWACEIADFFIKNKVGTVQMENLESMKRREDSYFNIRLRGFWPYAEMQNKIEFKLKQYGIVVRKVAPNNTSKTCSKCGHLNNYFNFEYRKKNKFPHFKCEKCNFKEDADYNAALNISNPKLKSTKGEP

SEQ ID NO: 2258 - protein, 726 aa, synthetic construct
SEVEFSHEYWMRHALTLAKRARDEREVPVGAVLVLNNRVIGEGWNRAIGLHDPTAHAEIMALRQGGLVMQNYRLIDATLYVTFEPCVMCAGAMVHSRIGRVVFGVRNSKRGAAGSLMNVLDYPGMNHRVETTEGILAEECAALLCDFYRMPRQVFNAQKKAQSTINSGSSSGGSSGSETPGTSESPTPESSGGIPGGSAKNTITKTLKLRIVRPYNSAEVEKIVADEKNNRERIALEKNKDKVKEACSKHLKVAAYCTTQVERNACLFCKARKLDDKFYQKLRGQFPDAVFWQEIGEIFRQLQKQAAEIYNQSLIELYYEIFIKGKGFANASSVEHYLSDVCYTRAAELFKNAAIASGLRGKVKSNFRLKELKNMRSGLPTTKSDNFPIPLVKQKGGQYAGFEISSHNDDFIIKIPFGRWQVKKEIDKYRPWEKFDFEQVRKSPKPISLLLSTRRRKRNKGWSKDEGTEAEIRKVMNGDYQTSYIEVKRGSKIGEKSAWMLNLSIDVPRIDKGVDPSIIGGIDVGVKSPLVCAINNAFGRYSISDNDLFHFNKKMFARRRILLKKNRHKRAGHGAKNKLKPITILTEKSKRFRKKLIERWACEIADFFIKNKVGTVQMENLESMKRKEDSYFNIRLRGFWPYAEMQDKIEFKLKQYGIEIRKVAPNNTSKTCSRCGHLNNYFSFEYRKKNKFPHFKCEKCNFKEDADYNAALNISNPKLKGTKEEL

SEQ ID NO: 2259 - protein, 726 aa, synthetic construct
GEVEFSHEYWMRHALTLAKRARDEREVPVGAILVLNNRVIGEGWNRAIGLHDPTAHAEIMALRQGGLVMQNYRLIDATLYVTFEPCVMCAGAMIHSRIGRVVFGVRNSKHGAAGSLVNVLSYPGMNHRVEITEGILADECAALLCDFYRMPRQVFNARKKTQSSINPGGSSDGSSGSETPGTSESATPESSGGSSGGSAKNTITKTLKLRIVRPYNSAEVEKIVADEKNNREKIALEKNKDKVKEACSKHLKMAAYCTTQVERNACLFCKARRLDDKFYRKLRGQFSDAVFWQEIGEIFRQLQKQAAEIYNQSLIELYYEIFIKGKGITNASRVEHYLSDVCYTRAAELFKNAAIASGLRNKIKSNFRLKELRNMRSGLPTTKSDNFPIPLVRQKGGQYTGFEISNHDGDFIIKIPFGRWQVKKEINKHRPWEKFDFEQVRKGPKPISLLLSTQRRKRNKGWSKDEGTEAEIRKVMNGDYQTSYIEVKRGSKIGEKSAWMLNLSIDVPKIDKGVDPSIIGGIDVGVKSPLVCAINNALSRYSISDNDLFHFNKKMFARRRILLKKNRHKRAGHGAKNKLKPISILTEKSKRFRKKLIERWACEIADFFIKNKVGTVQMENLEGMKRKEDSYFNIRLRGFWPYAEMQNKIEFKLKQYGIEVRKVTPNNTSKTCSKCGHLNNYFNFEYRKKNKFPHFKCEKCNFKENADYNAALNISNPKLKSTKEEP

SEQ ID NO: 2260 - protein, 726 aa, synthetic construct
SEVEFSHEYWMRHALTLAKRARDEREVPVGAILVLNNRVIGEGWNRAIGLHDPTAHAEIMALRQGGLVMQNYRLTDATLYVTFEPCVMCAGAMIHSRIGRVVFGVRNSKHGAAGSLMNVLNYPGMNHRVEITEGILVDECAALLCDFYRMPRQVFNARKKAQSSINPGGSSGGSSGSETPGASESASPKSSGGSPGSSAKNTITKTLRLRIVRPYNSAEVEKIVADEKNSREKIALEKNKDKVKEACSKHLRVAAYCTTQVDRNACLFCKARKLDDKFYQKLRGQFPDAVFWQEISEIFRQLQKQAAEIYNQSLIELYYEIFIKGKGIANASRVEHYLSDVCYTRAAELFKNAAIASGLRSKIKSNFRLKELRNMKSGLPTTMSDNFPIPLVKQKGGQYTGFEISNHNSDFIIKIPFGRWQVKKEIDKYRPWEKFDFEQVRKSPKPINLLLSTQRRKRSKGWSKDEGTEAEIRKVMNGDYQTSYIEVKRGSKIGEKSAWMLNLSIDVPKIDKGVDPSIIGGVDVGVKSPLVCAVNNALSRYSISDNDLFHFNKKMFARRRILLRKNRHKRAGHGARNKLKPITVLTEKSGRFRKKLIERWACEIAHFFIKNKVGTVQMENLESMKRREDSYFNIRLRGFWPYAEMQNKIEFKLRQYGIEIRKVAPNNTSKTCSKCGHLNNYFNFEYRKKNKFPHFKCEKCNFKENADYNAALNISNPKLKSTKEEP

SEQ ID NO: 2261 - protein, 726 aa, synthetic construct
SEVEFSHEYWMRHALTLAKRARDEREVPVGAILVLNNRVIGVGWNRAIGLHDPTAHAEIMALRQGGLVMQNYRLIDATLYVTFEPCVMCAGAMIHSRIGRVVFGVRNSKHGAAGSLVNVLNYPGMNHRVEITEGVLADECAGLLCDFYRMPRQVFSARKKAQSSINPGGSSGGSSGGKAPGTSESATLESSGGSSGGSAKNSITKTLKLRIVRPYNSAEVEKIVADEKNNREKIALEKNKDKVKEACSKHLKVAAYCTTQVERNACLFCKARRLDDKFYQKLRGQFPDAVFWQEIGEIFRQLQKQAAEIYNQSLVELYYEILIKGKGIANASSVEHYLSDVCYTRAAELFKNAAIASGLRNKIKSNFRLKELRNMRSGLPTTKSDNFPIPLVRQKGGQYTGFEISNHDGDFIIKIPFGRWQVKKEINKHRPWEKFDFEQVRKSPKPISLLLSTQRRKRNKGWSKDEGTEAEIRKVMNGDYRTSYIEVKRGSKIGEKSAWMLNLSIDVPKIDKGVDPGIIGGIDVGVKSPLVCAINNASSRYSISDNDLFHFNKKMFARRRILLKKNRHKRAGHGAKNKLKPITIMTEKSKRFRKKLIERWACEIADFFIKNKVGTVQMENLESMKRKEDSYFNIRLRGFWPYAEMQNKVEFKLKQYGIEIRKVAPNNTSKTCSKCGHLNNYFNFEYRKKNKFPHFKCEKCNFKENADYNAALNISNPKLKSTKEEP

SEQ ID NO: 2262 - protein, 726 aa, synthetic construct
SEVEFSHEYWMRHALTLAKRARDEREVPVGAVLVLNNRVIGGGWNRAIGLHDPTAHAEIMALRQGGLVMQNCRLVDATLYVTFEPCVMCAGAMIHSRIGRVVFGVRNSKRGAAGSLMNVLNYPGMNHRVEITEGILAGECAALLCDFYRMPRQVFNAQKKAQSTINSGGSSGGSSGSETPGTSESATPESSGGSSGSSAKNTITKTLKLRIVRPYNSAEVEKIVADEKNNREKIALEKNKDKVKEACSEHLKVAAYCTTQVERNACLFCKARKLDDRFYQKLRGQFPDAVFWQEIGEIFRQLQKQAAEIYNQSLIELYYEIFIKGKGFANASSVEHYLSDVCYTRAAELFKNAAIASGLRGKVKSNFRLKELKNMKSGLPTTKSDNFPIPLVKQKGGQYTGFEISSHNDDFIIKIPFGRWQVKKEIDKYRPWEKFDFEQVRKSPKPISLLLSTQRRKRNKGWSKDEGTEAEIRKVMNGDYQTSHIEVKRGSKTGEKSAWMLNLSIDVPKIDKGVDPSIIGGIDVGVKSPLVCAINNAFSRYSISDNDLFHFNKKMFARRRILLKKNRHKRAGHGAKNKLKPITILTEKSKRFRKKLIERWACEIADFFVKNKVGTVQMENLESMKRKEDSYFNIRLRGFWPYAEMQNKIEFKLKQNGIEIRKVAPNNTSKTCSKCGHLNNYFNFEYRKKNKFPHFKCEKCNFKENADYNAALNICNPKLKSTKEEP

SEQ ID NO: 2263 - protein, 726 aa, synthetic construct
SEVEFSHEYWMRHALTLAKRARDEREVPVGAILVLNNRVIGEGWNRAIGQHDPTAHAEIMALRQGGLVMQNYRLIDATLYVTFEPCVMCAGAMIHSRIGRVVFGVRNSKHGAAGSLVNVLNYPGMNHRVETTEGILAEECAALLCDFYRMPRQVFNAQKKAQSTINSGSSSGGSSGSETPGASESVTPKSSGGSSAGSTKNTITKTLKLRIVRPYNSAEVEKIVSDEKNNREKIALERNKDKVKEACSKHLKVAAYCTTQVERSACLFCKARKLDDKFYQKLRGQFPDAVFWQEIGEIFRQLQKQAAEIYNQSLIELYYEIFIKGKGFANASSVEHYLSDVCYTRAAELFKNAAIASGLRGKVKSNFRLKELRNMKSGLPTTKSDNFPIPLVKQKGGQYTGFEISSHNDDFIIKIPFGRWQMKKEIDRYRPWEKFDFEQVRKSPKPISLLLSTQRRKRNKGWSKDEGTEAEIRKVMNGDYQTSYIEVKRGSKTGERSAWMLNLSIDVPKIDKGADPSIIGGIDVGVKSPLVCAINNAFSRYSIGDNDLFRFNKKMFARRRILLKKNRHKRAGHGAKNKLKPISILTGKSERFRKKLIERWACEIADFFIKNKVGTVQMENLESMKRKEDSYFNIRLRGFWPYAEMQNKIEFKLKQYGIEIRKVAPNNTSRTCSKCGHLNNYFNFEYRRKYKFPHFKCEKCNFKEDADYNAALNISNPKLKSTKEGP

SEQ ID NO: 2264 - protein, 726 aa, synthetic construct; identical to SEQ ID NO: 684

SEQ ID NO: 2265 - protein, 726 aa, synthetic construct
SEVEFSHEYWMRHALTLAKRARDEREVPVGAILVLNNRVIGEGWNRAIGLHDPTAHAEITALRQGGLVMQNYRLIDATLYVTFEPCVMCAGAMIHSRIGRVVFGVRNSKHGAAGSLVNVLNYPGMNHRVEITEGILADECAALLCDFYRMPRQVFNARKKAQPSINPGGSSGGSSGSETPGTSESATPESSGGNSGGSAKNTITKTLTLRIVRPYNSAEVEKIVADEKNNREKIALEKNKDKVKEACSEHLKVATYCTTRVERNACPFCKARKLDDKFYQKLRGQFPDAVFWQELGEILRQLQKQAAEIYNQSLIELYYEIFIKGRGFANASSVEHYLSDVCYTRAAELFKNAAIASGLRGKVKSNFRLKELKNMKSGLPTTKSDNFPIPLVKQKGGQYTGFEISSHNDDFIIKIPFGRWQVKEEIDKYRPWEKFDFEQVRKSPKPISLLLSTQRRKRNKGWSKDEGTEAEIRKVMNGDYQTSYIEVKRGSRTGEKSAWMLNLSIDVPKIDKGVDPSIIGGIDVGVKSPLVCAINNAFSRYSISDNDLFRFNKKMFARRRILLKKNRHKRAGHGAKNKLKPISILTGKSERFRKKLIERWACEIADFFTKNKVGTVQMENLESMKRKEDSYFNIRLRGFWPYAEMQNKIEFKLKQYGIEIRKVAPNNTSKTCSKCGHLNNYFNFEFRKKNKFPHFKCEKCNFKEDADYNAALNISNPKLKSTKEEP

SEQ ID NO: 2266 - protein, 726 aa, synthetic construct
SEVEFSHEYWMRHALTLAKRARDEREVPVGAVLVLNNRVIGEGWNRAIGLHDPTAHAEIMALRQGGLVMQNYRLTDATLYVTFEPCVMCAGAMIHSRIGRVVFGVRNSKHGAAGSLVNVLNYPGMNHRVEITEGILADECAALLCDFYCMPRQVFNAQKRAQSSINSGGSSGGSSGSETPGTSESATPESSGGGSSGSAKNTITKTLQLRIVRPYNSAEVEKIVADEKNNREKIALEKNKDKVKEACSEHLKVAAYCTTQVERNACLFCKARRLDDKFYQKLRGQFPDAVFWQEIGEIFRQLQKQAAEIYNQSLVELYYEIFIKGKGIANASSVEHYLSDVCYTRAAELFKNAAIASGLRNKIKSNFRLKELRNMKSGLPTTKSDNFPIPLVRQKGGQYTGFEISNHNGDFIIKIPFGRWQVKKEISKHRPWEKFDFEQVRKSPKPISLLLSTQRRKRNKGWSKDEGTEAEIRKVMNGDYQTSYIEVKRGSKIGEKGAWMLNLSIDVPKIDKGVDPSIIGGIDVGVKSPLVCAINNAFSRYSISDNDLFHFNKKMFARRRILLKKNRHKRAGHGAKNKLKPLTILTGKSKRFRKKLIERWACEIADFFIKNKVGTVQMENLESMKRKEDSYFNIRLRGFWPYAEMQNKIEFKLKQYGIKIRKVAPNNTSKTCSKCGHLNNYFSFEYRKKNKFPHFKCEKCNFKEDADYNAALNISNPNLKSTKEEP

SEQ ID NO: 2267 - protein, 726 aa, synthetic construct
SEVEFSHEYWMRHALTLAKRARDEREVPVGAILVLNNRVIGVGWNRAIGLHDPTAHAEIMALRQGGLVMQNYRLIDATLYVTFEPCVMCAGAMIHSRIGRVVFGVRNSKHGAAGSLVNVLNYPGMNHRVEITEGILADECAALLCDFYRMPHQVFNARKRAQSSINSGGSSGSSSGSETPGSSESATPESSGGGSSGSAKNTITKTLQLRIVRPYNSAEVEKIVADEKSNREKVALEKNKDKVKEACSKHLKVAAYCTTQVERNACLFCKARKLDDKFYQKLRGQFPDAVFWQEIGEIFRQLQKQAAEIYNQSLVELYYEIFIKGKGIANASSVEHYLSDVCYTRAAELFKNAAIASGLRNKVKSNFRLKELRNMKSGLPTTKSDNFPIPLVRQKGGQYTGFEISNHNDDFIIKIPFGRWQAKKEIDKYRPWEKFDFEQVRKSPKPISLLLSTRRRKRNKGWSKDEGTEAEIRKVMNGDYQTSYIEVKRGSKIGEKSAWMLNLSIDVPKIDKGVDPSIIGGIDVGVKSPLVCAINNALSRYSISDNDLFHFNKKMFARRRILLRKNRHKRAGHGARNKLKPITVLTEKSERYRKKLIERWACEIANFFIKNKVGTVQMENLESMKRREDSYFNIRLRSFWPYAEMQNKIEFKLKQYGIEIRKVAPNNTSKTCSRCGHLNNYFNFEFRKRNKFPHFKCEKCNFREDADYNAALNISSPKLKSTKEEP

SEQ ID NO: 2268 - protein, 726 aa, synthetic construct
SEVEFSHEYWMRHALTLAKRARDEREVPVGAILVLNNRVIGEGWNRAIGLHDPTAHAEIMALRQGGLVMQNYRLIDATLYVTFEPCVMCAGAMIHSRIGRVVFGVRNSKHGAAGSLVNVLNYPGMNHRVETTEGILAGECAALLCDFYRMPRQVFNAQKKAQSTINSGGSSGGSSSSETPGTSGSATPEGSGGSSGGSAKSTITKTLKLRIVRPYNSAEVEKIVADEKNNREKIALEENKDKVKEACSKHLKVASYCTTQVARNACLFCKARKLDDKFYQRLRGQFPDAVFWQELGEIFRQLQKQAAEIYNQSLIELYYEIFIKGKGFANASSVEHYLSDVCYTRAAELFKNAAIASGLRGKVKSNFRLKELKNMKSGLPTTKSDNFPIPLVRQKGGQYTGFEISSHNDDFIIKIPFGRWQVRKEIDKYRPWEKFDFEQVRRSPKPISLLLSTQRRKKNKGWSKDEGTEAEIRKVMNGDYQTSYIEVKRGSKIGEKSAWMLNLSIDVPKIDKGVDPSIVGGIDVGVKSPLVCAIDNALSRYSISDNDLFHFNKKMFARRRILLKKNRHRRAGHGAKNKLKPISILTEKSKRFRKKLIERWACEIADFFIKNKVGTVQMENLESMKRKEDSYFNIRLRGFWPYAEMQNKIEFKLKQYGIEIRKVAPNNTSKTCSKCGHLNNYFNFEYRKKNKFPHFKCEKCNFKENADYNAALNICNPKLKSTKEEP

SEQ ID NO: 2269 - protein, 726 aa, synthetic construct
SEVEFSHEYWMRHALTLAKRARDGREVPVGAVLVLNNRVIGEGWNRAIGLHDPTAHAEIMALRQGGLVMQNYRLIDATLYVTFEPCAMCAGAMVHSRIGRVVFGVRNSKRGAAGSLMNVLNYPGMDHRVEITGGILADECAALLCDFYRMPRRVFNAQKKAQSSINSGGSSGGSSGSETPSTSESATPESSGGSSGGSAKNTITKTLQLRIVRPYNSAEVEKIVADEKNNREMIALEKNRDKVKEACSKHLKVAAYCTTQVERNACLFCKARRLDDKFYQKLRGQFPDAVFWQEIGEIFRQLQKQAAEIYNQSLIELYYEIFIKGKGFANASSVEHYLSDVCYTRAAELFKNAAIASGLRGKVKSNFRLKELKNMKSGLPTTKSDNFPIPLVRQKGGQYTGFEISGHNDDFIIKIPFGRWQVKKEIDKYRPWEKFDFEQVRKSPKPISLLLSTQRRKRNKGWSKDEGTEAEIRKVMNGDYQTSYIEVKRGSKIGEKSAWMLNLSIDVPKIDKGVDPSIIGGIDVGVKSPLVCAIDNAFSRYSISDNDLFHFNKKMFARRRILLKKNRHKRAGHGAKNKLKPISILTEKSKRFRKKLIERWACEIADFFIKNKVGTVQMENLESMKRKEDSYFNIRLRGLWPYAEMQNKIEFKLKQYGIKIRKVAPNNTSKTCSKCGHLNNYFNFEYRKKNKFPHFKCEKCSFEENADYNAALNISNPKLKSTKEEP

SEQ ID NO: 2270 - protein, 726 aa, synthetic construct
SEVEFSHEYWMRHALTLAKRARDEREVPVGAVLVLNNRVIGEGWNRAIGLHDPTAHAEIMALRQGGLVMQNYRLIDATLYVTFEPCVMCAGAMVHSRIGRVVFGVRNSKRGAAGSLMNVLDYPGMDHRVGITEGILADECAALLCDFYRMPRQVFNAQKKAQSSINPGGSSGGSSGSETPGASESVTPKSSGGSSAGSTKNTITKTLKLRIVRPYNSAEVEKIVADEKNSREKIALEKNKDKVKEACSKHLKVAAYCTTQVERNACLFCKARKLDDKFYQKLRGQFPDAVFWQEISEIFRQLQKQAAEIYNQSLIELYYEIFIKGKGFANASSVEHYLSDVCYTRAAELFKNAAIASGLRNKVKSNFRLKELRSMKSGLPTTKSDNFPIPLVRQKGGQYTGFEISNHNGDFIIKIPFGRWQAKKEIDKYRPWEKFDFEQVRRSPKPISLLLSTQRRKKNKGWSKDEGTEAEIRRVMNGDYQTSYIEVKRGSKIGEKSAWMLNLSIDVPKVDKGVDPSIIGGIDVGVKSPLVCAVNNSFSKYSICDNDLFRFNKKMFARRRILLKKNRHKRAGHGAKNKLKPITILTKKSERFRKKLIERWACEVADFFIKNKVGTVQMENLESMKRREDSYFNIRLRGFWPYAEMQNKIEFKLKQYGIEIRKVAPSNTSKTCSRCGHLNNYFNFEFRKRNKFPHFKCEKCNFKENADYNAALNISNPKLKSTKEEP

SEQ ID NO: 2271 - protein, 725 aa, synthetic construct
SEVEFSHEYWMRHALTLAKRARDEREVPVGAVLVLNNRVIGEGWNRAIGLHDPTAHAEIMALRQGGLVTQNYRLIDATLYVTFEPCVMCAGAMIHSRIGRVVFGVRNSKHGAAGSLMNVLNYPGMNHHVEITEGILVDECAALLCDFYRMPRQVFNARKKAQSSINPGGSFGGSSGSETPGTSESATLESSGGSSGGSAKNTITKTLKLRIVRPYNSAEVEKIVADEKDNREKIALEKNKDKVKEACSKHLKVAAYCTTQVERNACLFCKARKLDDMFYQKLRGQFPDAVFWQEIGEVFRQLQKQAAEIYNQSLIELYYEIFIKGKGLANASSVEHYLSDVCYARAAELFKNAAIASGLRGKVKSNFRLKELKNMKSGLPTTKSDNFPIPLVKQKGGKYAGFEISSHNDDFIIKIPFGRWQVKKEIDKYRPWEKFDFEQVRKSPKPISLLLSTQRRKRNKGWSKDEGTEAEIRKVMSGDYQTSYIEVKRGSKIGEKSAWMLNLSIDVPKIDKGVDPSIIGGIDVGVKSPLVCAINNAFSRYSIGDNDLFHYNKKMFARRRILLKKNRHKRAGHGARNKLKPITVLTEKSKRFRKKLIERWACEIANFFIKNKVGTVMENLESMKRKEDSYFNIRLRGFWPYAEMQNKIEFKLKQYGIEIRKVAPNNTSKTCSKCGHLNNYFNFEYRKKNKFPHFKCEKCNFKENADYNAALNISNPMLKSTKEEP

SEQ ID NO: 2272 - protein, 726 aa, synthetic construct
SEVEFSHEYWMRHALTLARRARDEREVPVGAILVLNNRVIGEGWNRAIGLHDPTAHAEIMALRQGGLVMQNYRLVDATLYVTFEPCVMCAGAMIHSRIGRVVFGVRNNKHGAAGSLMNVLNYPGMNHRVEITEGILADECAALLCDFYRMPRQVFNARKKAQSSINPGGSSGGSSGSETPGTSESATPESSGGSSGSSAKNTITKTLKLRIVRPYNSAEVEKIVADEKNNREKIALEKNKDKVKEACSKHLKVAAYCTTQVGRNACLFCKARRLDDKFYQKLRGQFPDAVFWQEIGEIFRQLQKQAAEVYNQSLVELYYEILIKGKGIANASSVEHYLSDVCYTRAAELFKNAAIASGLRNKIKSNFRLKELRNMKSGLPTTKSDNFPIPLVRQKGGQYTGFEISNHDGDFIIKIPFGRWQVKKEIDKYRPWEKFDFEQVRKSPKPISLLLSTQRRKRNKGWSKDEGTEAEIRKVMNGDYQTSYIEVKRGSKIGEKSAWMLNLSIDVPKIDKGVDPSIIGGIDVGVKSPLVCAISNAFSRYSISDNDLFHFNKKMFARRRILLKKNRHRRAGHGAKNKLKPITILTEKSVRFRKKLIERWACEIADFFIKNKVGTVQMENLESMKRKEDSYFNIRLRGFWPYAEMQNKIEFKLKQYGIEIRRVAPNNTSRTCSKCGHLNNYFNFEYRKKNKFPHFKCEKCNFKENADYNAALNISNPKLKSTKEEP

SEQ ID NO: 2273 - protein, 726 aa, synthetic construct
SEVEFSHEYWMRHALTLAKRARDEREVPVGAVLVLNNRVIGEGWNRAIGLHDPTAHAEIMALHQGGLVMQNYRLIDATLYVTFEPCVMCAGAMIHSRIGRVVFGARNSKRGAAGSLMNVLSYPGMNHRVEITEGILADECAALLCDFYRMPRRVFNARKKAQSSINSGGSSGGGSGSDTPSTSESTTPESSGGSSGGPAKNTITKTLKLRIVRPYNSAEVEKIVADEKNNREKTALEKNKDKVKEACSKHLKVAAYCTTQVERNACLFCKARKLDDKFYQKLRGQFPDAVFWQEVGEIFRQLQKQAAEIYNQSLIELYYEIFIKGKGFANASSVEHYLSDVCYTRAAELFRNAAIASGLRGKVKSNFRLKELKNMKSGLPTTKSDNFPIPLVKQKGGQYTGFEISSHNDDFIIKIPFGRWQVKKEIDKYRPWEKFDFEQVRKSPKPISLLLSTQRRKRNKGWSKDEGTEAEIRKVMNGDYQTSYIEVKRGSKTGEKSAWMLNLSIDVPKIDKGVDPSIIGGIDVGVKSPLVCAINNAFNRYSISDNNLFHFNKKMFARRRILLKKNRHKRAGHGAKNKLRPISILTEKSERFRKKLIERWACEIADFFIRNKVGTVQMENLEGMKRKEDSYFNIRLRGFWPYAEMQNKIEFKLKQYGIEVRKVAPNNTSKTCSKCGHLNNYFNFEYRKKNKFPHFKCEKCNFKENADYNAALNISNPKLKSTKEEP

SEQ ID NO: 2274 - protein, 726 aa, synthetic construct
SEVEFSHEYWMRHALTLAKRARDEREVPVGAILVLNNRVIGEGWNRAIGLHDPTAHAEIMALRQGGLVMQNYRLIDATLYVTFEPCVMCAGAMIHSRIGRVVFGVRNSKHGAAGSLMDVLNYPGMNHRVEITEGILADECAALLCDFYRMPRQVFSARKKAQSSINPGGSSGGSSGSKTPGTSESATPESSGGSSGGSAKNSITKTLKLRIVRPYNSAEVEKIVADEKNNREKIALEKNKGKVKEACSKHLKVATYCTTQVERNACLFCKARKLDDKFYQKLRGQFPDAVFWQEIGEIFRQLQKQAAEIYNQSLIELYYEIFIKGKGFANASSVEHYLSGVCYTRAAELFKNAAIASGLRGKVKSNFRLKELKNMRSGLPTTKSDNFPIPLVKQKGGQYTGFEISSHNDDFIIKIPFGRWQEKKEIDKYRPWEKFDFEQVRKSPKPISLLLSTQRRKRNKGWSKDEGTEAEIRKVMNGDYQISYIEVKRGSKIGEKSAWTLNLSVDVPKIDRGVDPSIIGGIDVGVKSPLVCAINNALSRYSISDNDLFHFNKKVFARRRILQKKNRHRRAGHGAKNKLKPITILTEKSKRFRKKLIERWACEIADFFIKNKVGIVQMENLESMKRREDSYFNIRLRGFWPYAEMQNKIEFKLKQYGIEIRKVAPNNTSKTCSRCGHLNNYFNFEYRRKNKFPHFKCEKCNFKEDADYNAALNISNPKLKSTKEEP

SEQ ID NO: 2275 - protein, 726 aa, synthetic construct
SEVEFSHEYWMRHALTLAKRARDEREVPVGAVLVLNNRAIGVGWNRAIGLHDPTAHAEIMALRQGGLVMQNYRLVDATLYVTFEPCIMCAGAMIHSRIGRVVFGVRNSKRGAAGSLMNVLNYPGMNHRVEITEGILAGECAALLCDFYRMPRQVFNAQKKAQSSISSGGSSGGSSGSETPGASGSVTPKSSGGSSAGSTKDTVTKTLMLRIVRPYNSAEVEKIVADEKNSREKIALEKNKDKVKEACSEHLKVAAYCTTQVERNACLFCKARKLDDKFYQKLRGQFPDAVFWQELGEIFRQLQKQAAEIYNQSLIELYYVIFIKGKGTANASSVEHYLSDVCYTRAAALFKNAAIASGLRNKIKSNFRLKELRNMKSGLPTTKSDNFPIPLVKQKGGQYTGFEISSHNDDFIIKIPFGRWQVKKETDKYRPWEKFDFEQVRKSPKPISLLLSTQRRKRNKGWSKDEGTEAEIRKVMNGDYQTSYIEVKRGSKIGEKSAWMLNLSIDVPKIDKGVDPSIIGGIDVGVKSPLVCAINNALSRYSISDNDLFHFNKKMFARRRILLRKNRHKRAGHGARNKLKPITVLTEKSERFRKKLIERWACEIANFFIKNKVGTVQMENLESMKRREDSYFNIRLRGFWPYAEMQSKIEFKLKQYGIEVRRVAPNNTSKTCSKCGHLNNYFNFEFRKKNKFPHFKCEKCNSKEDADYNAALNISNPKLKSTKEEP

SEQ ID NO: 2276 - protein, 726 aa, synthetic construct
SEVEFSHEYWMRHALALAKRARDEREVPVGAVLVLNNRVIGEGWNRAIGLHDPTAHAEIMALRQGGLVMRNYRLTDATLYVTFEPCVMCAGAMIHSRIGRVVFGVRNSKRGAAGSLMNVLNYPGMNHCVEITEGILVDECAALLCDFYRMPRQVLNAQKKAQSSINSGGSSGGSSGSETPGTSESATPESSGGGSSGSAKNTITKTLQLRIVRPYNSAEVEKIVADEKNSREKIALEKNKGKVKEACSEHLKVAAYCTTQVERNACLFCKARKLDDRFYQKLRGQFPDAVFWQEIGEIFRQLQKQAAEIYNQSLIELYYEIFIKGKGFANASSVEHYLSDVCYTRAAELFKNAAIASGLRGKVKSNFRLKELKSMKSGLPTTKSDNFPIPLVKQKGGQYTGFEVSSHNDDFIIKIPFGRWQVKKEIDKYRPWEKFDFEQVRKSPRPISLLLSTQRRKRNKGWSKDEGTEAEIRKVMNGDYQTSYIEVKRGSKIGEKSAWMLNLSIDVPKIDKGVDPSIIGGIDVGVKSPLVCAINNALSRYSISDNDLFHFNKKMFARRRILLRKNRHKRAGHGAKNKLKPITIMTEKSKRFRKKLIERWACEIADFFIKNKVGTVQMENLESMKRKEDSYFNIRLRGFWPYAEMQNKIEYKLKQYGIEIRRVAPNNTSRTCSKCGHLNNYFNFEYRRKYKFPHFKCEKCNFKEDADYNAALNISNPKLKSTKEEP

SEQ ID NO: 2277 - protein, 726 aa, synthetic construct; identical to SEQ ID NO: 684

SEQ ID NO: 2278 - protein, 726 aa, synthetic construct
SEVEFSHEYWMRHALTLAKRARDEREVPVGAILVLNNRVIGEGWNRAIGLHDPTAHAEIMALRQGGLVMQNYRLIDATLYVTFEPCVMCAGAMIHSRIGRVVFGVRNNKHGAAGSLVNVLNYPGMNHRVEITEGILADECAALLCDFYRMPRQVFNARKKAQSSINPGGSSGGSSGSETPGTSESATPESSGGSSGSSAKNTITKTLKLRIVRPYNSAEVEKIVADEKNNREKIALEKNKDKVKEACSKHLKVAAYCTTQVERNACLFCKARRLDDKFYQKLRGQFPDAVFWQEIGEIFRQLQKQAAEVYNQSLVELYYEILIKGKGIANASSVEHYLSDVCYTRAAELFKNAAIASGLRNKIKSNFRLKELRNMKSGLPTTKSDNFPIPLVRQKGGQYTGFEISNHDGDFIIKIPFGRWQVKKEINKHRPWEKFDFEQVRKSPKPISLLLSTQRRKRNKGWSKDVGTEAEIRKVMNGDYQTSYIEVKRGSKVGERSAWMLNLSIDVPKIDKGVDPSIIGGIDVGVKSPLVCAINNALSRYSISDNDLFHFNKKVFARRRILLKKNRHKRAGHGTKNKLKPITILTEKSGRFRKKLIERWACEIANFFIKNKVGTVQMENLESMKRKEDSYFNIRLRGFWPYAEMQNKIEFKLKQYGIKIRKVAPNNTSKTCSKCGHLNNYFSFEYRKKNKFPHFKCEKCNFKEDADYNAALNISNPKLKSTKEEP

SEQ ID NO: 2279 - protein, 726 aa, synthetic construct
SEVEFSHEYWMRHALTLAKRARDEREVPVGAVLVLNNRVIGEGWNRAIGLHDPTAHAEIMALRQGGLVMQNYRLIDATLYVTFEPCVMCAGAMIHSRIGRVVFGVRNSKHGAAGSLVNVLNYPGMNHRVEITEGILAGECAALLCDFYRMPHQVFNVRRKAQSSINPGGSSGGSSGSETPGTSESPTPESPGGSSGGSAKNTITKTLKLRIVRPYNSTEVEKIVADEKNNREKIALEKNKDKVKEACSKHLKVAAYCTTQVERNACLFCKARKLDDKFYQKLRSQFPDAVFWQELGEILRQLQKQAAEIYNQSLIELYYEIFIKGRGFANASSVEHYLSDVCYTRAAELFKNAAIASGLRGKVRSNFRLKELKNMKSGLPTTKSDNFPIPLVKQKGGQYTGFEISNHNSDFIIKIPFGRWQVKKEIDKYRPWEKFDFEQVRKSPKPISLLLSTQRRKRNRGWSKDEGTEAEIKKVMNGDYQTSYIEVKRGSKTGEKSAWMLNLSIDVPKIDKGVDPCIIGGIDVGVKSPLVCAINNASSRYSISDNDLFHFNKKMFARRRILLKKNGHKRAGHGTKNKLKPITIMTEKSKRFRKKLIERWACEVADFFIKNKVGTVQMENLESMKRKEDSYFNIRLRGFWPYAELQNKIEFKLKQYGIVVRKVAPNNTSKTCSKCGHLNNYFNFEYRKMNKFPHFKCEKCNFKENADYNAALNISNPKLKSIKEEP

SEQ ID NO: 2280 - protein, 726 aa, synthetic construct
SEVEFSHEYWMRHALTLAKRARDEREVPVGAVLVLNNRVIGEGWNRTIGLHDPTAHAEIMALRQGGLVMQNYRLTDATLYVTFEPCVMCAGAMIHSRIGRVVFGVRNSKRGAAGSLMNVLNYPGMNHCVEITEGILVDECAALLCDFYRMPRQVLNAQKKAQSSISSGGSSGGSSGSETPGASESVTPKSSVGSSAGSTKNTITKTLKLRIVRPYNSAEVEKIVADEKNNRERIALEKNKDKVKEACSKHLKVAAYCTTQVERNACLFCKARKLDDKFYQKLRGQFPDAVFWQEVGEIFRQLQKQAAEIYNQSLIELYYEIFIKGKGFANASSVEHYLSDVCYTRAAELFKNAAIASGLRGKVKSNFRLKELKNMKSGLPTTKSDNFPIPLVKQKGGQYTGFEISNHDGDFIIKIPFGRWQVKKEINKHRPWEKFDFEQVRKSPKPISLLLSTQRRKRNKGWSKDEGTEAEIRKVMNGDYQTSYIEVKRGSKIGEKSAWMLNLSIDVPKIDKGVDPGIIGGIDVGVKSPLVCAINNASGRYSISDNDLFHFNKKMFARRRILLKKNRHKRAGHGAKNKLKPITIMTEKSKRFRKKLIERWACEIADFFIKNKVGTVQMENLESMKRKEDSYFNIRLRGFWPYAEMQNKIEFKLKQYGVEIRKVAPNNTSKTCSKCGHLNNYFSFEYRKKNKFPHFKCEKCNFKEDADYNAALNISNPKLKSTKEEP

SEQ ID NO: 2281 - protein, 726 aa, synthetic construct
SEVEFSHEYWMRHALALAKRARDEREVPVGAVLVLNNRVIGEGWNRAIGLHDPTAHAEIMALRQGGLVLQNYRLVDATLYVTFEPCVLCAGAMVHSRIGRVVFGARNSKRGAAGSLMNILNYPGMNHRVEITEGILADECAALLCDFYRMPRQVFNAQKKAQSSINSGGSSGGSSGSETPSTSESATPESSGGSSGGSAKNTITKTLKLRIVRPYNSAVVEKIVADEKNNREKIALEKNKDKVKEACSEHLKVAAYCTIQVERNACLFCKARKLDDRFYQKLRGQFPDAVFWQETGEIFRQLQRQAAEIYNQSLIELYYEIFIKGKGFANASSVEHYLSDVCYTRAAELFKNAAIASGLRGKVKSSFRLKELKNMKSGLPTTKSDNFPIPLVKQKGGQYTGFEISSHNDDFIIKIPFGRWQVKKEIDKYRPWEKFDFEQVRKSPKPISLLLSTQRRKRNKGWGKDEGTEAEIRKVMNGDYQTSYIEVKRGSKIGEKSAWMLNLSIDVPKIDKGVDPSIIGGIDVGVKSPLVCAINNAFSRYSISDNDLFRFNKKMFARRRILLKKSKHKRAGHGAKNKLKPITILTEKSGRFRKKLIERWACEIADFFIKNKVGTVQMENLESMKRKEDSYFNIKLRGFWPYAEMQNKIEFKLKQYGIEIRKVAPNNTSKTCSKCGHLNNYFNFEYRKTNKFPYFKCEKCNFKEDADYNAALNISNPKLKSTKEEP

SEQ ID NO: 2282 - protein, 726 aa, synthetic construct
SEVEFSHEYWMRHALTLAKRARDEREVPVGAVLVLNNRVIGEGWNRTTGLHDPTAHAEIMALRQGGLVMRNYRLTDATLYVTFEPCVMCAGAMIHSRIGRVVFGVRNSKRGAAGSLMNVLNYPGMNHCVEITEGILVDECAALLCDFYRMPRQVLNAQKKAQSSVSSGGSSGGSSGSETPGASGSVTPKSSVGSSAGSTKNTITKTLKLRIVRPYNSAEVEKIVADEKNNREKIALEKNRDKVKEACSEHLKVAAYCTTQVERNACLFCKARRLDDKFYQKLRGQFPDAVFWQEIGEIFRQLQKQAAEIYNQSLVELYYEILIKGKGIANASSVEHYLSDVCYTRAAKLFKNAAIASGLRNKIKSNFRLKELRNMKSGLPTTKSDNFPIPLVRQKGGQYTGFEISNHDGDFIIKIPFGRWQVKKEINKHRPWEKFDFEQVRKSPKPISLLLSTQRRKRNKGWSKDEGTEAEIRKVMNGDYQISYIEVKRGSKIGEKSAWMLSLSVDVPKIDKGVDPSVIGGIDVGVKSPLVCAINNALSRYSISDNDLFHFNKKMFARRRILLRNNRHKRAGHGAKSKLKPITILTEKGERFRKKLIERWACEIANFFIKNKVGTVQIENLESMKRKEDSYFNIRLRGFWPYAEMQNKIEFKLKQYGIEIRKVAPNNTSKTCSKCGHLNNYFNFEYRKMNKFPHFKCEKCNFKENADYNAALNISNPKLKSTKEEP

SEQ ID NO: 2283 - protein, 726 aa, synthetic construct; identical to SEQ ID NO: 684

SEQ ID NO: 2284 - protein, 726 aa, synthetic construct
SEVEFSHEYWMRHALTLAKRARDEREVPVGAILVLNNRVIGEGWNRAIGLHDPTAHAEIMALRQGGLVMQNYRLIDATLYVTFEPCVMCAGAMIHSRIGRVVFGVRNNKHGAAGSLVNVLNYPGMNHRVEITEGILADECAALLCDFYRMPRQVFNARKKAQSSINPGGSSGGSSGSETPGTSESATPESSGGSSGSSAKNTITKTLKLRIVRPYNSAEVEKIVADEKNNREKIALEKNKDKVKEACSKHLKVAAYCTTQVERNACLFCKARRLDDKFYQKLRGQFPDAVFWQEIGEIFRQLQRQAAEIYNQSLIELYYEIFIKGKGITNASRVEHYLSDVCYTRAAELFKNAAIASGLRSKVRSNFRLKELKNMKSGLPTTKSDNFPIPLVKQKGGQYTGFEISSHNSDFIIKIPFGRWQEKEEIDKYRPWEKFDFEQVRRSPKPISLLLSTQRRKKNKGWSKDEGTEAEIRRVMNGDYQTSYIEVKRGSKIGEKSAWMLNLSIDVPKIDKGVDPSIIGGIDVGVKSPLVCAINNAFSRYSISDNDLFHFNKKMFARRRILLKKNRRRRAGHGAKNKLKPITILTEKSVRFRKKLIERWACEIADFFIKNKVGTVQMENLESMKRKEDSYFNIRLRGFWPYAEMQNKIEYKLKQYGIKIRKVAPNNTSKTCSKCGHLNNHFSFEYRKKNKFPHFKCEKCNLKEDADYNAALNISNPKLKSTKEEP

SEQ ID NO: 2285 - protein, 726 aa, synthetic construct
SEVEFSHEYWMRHALTLAKRARDEREVPVGAVLVLNNRVIGEGWNRAIGLHDPTAHAEIMALRQGGLAMQNYRLVDATLYVTFEPCVLCAGAMVHSRIGRVVFGVRNSKRGAAGSLMNVLNHPGMNHRVEITGGILADECAALLCDFYRMPRQVFNAQKKARSNINSGGSSGGSSGSETLGTSESATPESSGGSPGGSAKNTITKTLKLRIVRPYNSAEVEKIVADEKNNRERIALEKNKDKVKEACSKHLKVAAYCTTQVERNACLFCRARRLDDKFYQKLRGQFPDAVFWQEIGEIFRQLQKQAAEIYNQSLIELYYEIFIKGKGFANASSTEHYLSDVCYTRAAELFKNAAIASGLRGKVKSNFRLKELKNMKSGLPTTKSDNFPIPLVKQKGGQYTGFEISSHNDDFIIKIPFGRWQVKKEIDRYRPWEKFDFEQVRKSPKPISLLLSTQRRKRNKGWSKDEGTEAEIRKVMNGDYQTSYIEVKRGSKIGEKSAWMLSLSIDVPKIDKGVDPSTIGGIDVGVKSPLVCAINNAFCRYSISDNDLFHFNKKMFARRRILLKKSRHKRAGHGAKNKLKPISVLTERSKRFRKKLIERWACEIADFFVKNKVGTVQMENLESMKRKEDSYFNIRLRGFWPYAEMQNKIEFKLKQYGIEIRKVAPNNTSKTCSKCGHLNNYFNFEYRKRNKFPHFKCEKCNFKENADYNAALNISNPKLKSTKEEP

SEQ ID NO: 2286 - protein, 726 aa, synthetic construct
SEVEFSHEYWMRHALTLAKRARDEREVPVGAILVLNNRVIGEGWNRAIGLHDPTAHAEIMALRQGGLVMQNYRLIDATLYVTFEPCVMCAGAMIHGRIGRVVFGVRNSKRGAAGSLMNVLNHPGMSHRVEITGGILADECAALLCDFYRMPRQVFNAQKKARSNINSGGSSGGSSGSETLGTSESATPESSGGSSGGSAKNTITKTLKLRIVRPYNSAEVEKIVADEKNNREKIALEKNKDKVREACSKHLKVAAYCTTQVERNACLFCKARRLDDKFYQKLRGQFPDAVFWQEIGEIFRQLQKQAAEIYNQSLVELYYEIFIKGKGIANASSVEHYLSDVCYTRAAELFKNAAIASGLRNKIKSNFRLKELRNMKSGLPTTKSDNFPIPLVRQKGGQYTGFEISNHNGDFIIKIPFGRWQVKKEISKHRPWEKFDFEQVRKGPKPISLLLSTQRRKRNKGWSKDEGTEAEIRKVMSGDYQTSYIEVKRGSKIGEKSAWMLNLSIDVPKIDKGVDPSIIGGIDVGVKSPLVCAINNAFSRYSISDNDLFRFNKKMFARRRILLKKNRHKRAGHGAKNKLKPITTLTEKSRRFRKKLIERWACEIADFFIKNKVGTVQMESLESMKRKEDSYFNIRLRGFWPYAEMQNKIEFKLKQYGIEIRKVAPNNTSKTCSRCGHLNNYFNFEYRRKNKFPHFKCERCNFKENADYNAALNISNPKLKSTKEEP

SEQ ID NO: 2287 - protein, 726 aa, synthetic construct
SEDEFSHEYWMRHALTLAKRARDGREVPVGAVLVLNNRVIGEGWNRAIGLHDPTAHAEIMALRQGGLVMQNYRLTDATLYVTFEPCVMCAGAMIHSRIGRVVFGVRNSKRGAAGSLMNVLNHPGMNHCVEITEGILVDECAALLCDFYRMPRQVLNAQKKAQSSISPSGSSGGSSGSETPGASESVTPKSSGGSSGGSAKNTITKTLKLRIVRPYNSAEVEKIVADEKNNREKIALEKNKGKVKEACSKHLEVAAYCTTQVERNACLFCKARKLDDKFYQKLRGQFPDAVFWQELGEIFRQLQRQAAEIYNQSLIELYYEIFIKGKGFANASSVEHYLSDVCYTRAAELFKNAAIASGLRGKVKSNFRLKELKNMKSGLPTTKSDNFPIPLVKQKGGQYTGFEISSHNDDFIIKIPFGRWQVKEEIDKYRPWEKFDFEQVRKSPKPISLLLSTQRRQKNKGWSKDEGTEAEIRRVMNGDYQTSYIEVKRGSKIGEKSTWMLNLSIDVPKIDKGVDPSIVGGIDVGVKSPLVCAINNSFSRYSICDNDLFRFNKKMFARRRILLRKNRHKRAGHGAKNKLKPITILTKKSERFRKKLIERWVCEVADFFIKNKVGTVQMENLESMKRKEDSYFNIRLRGFWPYAEMQNRIELKLKQYGIEIRRVAPNNTSKTCSKCGHLNNYFNFEYRRKNRFPHFKCEKCNFKENADYNAALNISNPKLKSTKEEP

SEQ ID NO: 2288 - protein, 726 aa, synthetic construct
SEVEFSHEYWMRHALTLAKRARDEREVPVGAVLVLNNRVIGEGWNRVIGLHDPTAHAEIMALRQGGLVMQNYRLTDATLYVTFEPCVMCAGAMIHSRIGHVVFGVRNSKRGAAGSLMNVLNYPGMNHCVEITEGILVDECAALLCDFYRMPRQVLNAQKKAQSSISSGGSSGGSSGSVTPGASGSVTPKSSGGSSAGSTKDTITKTLKLRIVRPYNSAEVEKIVADEKNNREMIALEKNKDKVKEACSEHLKVAAYCTAQVERSACLFCKARKLDDKFYQKLRGQFPDAVFWQEIGEIFRQLQKQAAEIYNQSLIELYYEIFIKGKGFANASSVEHYLSDVCYTRAAELFKNAAIASGLRGKVKSNFRLKELKNMKSGLPTTKSDNFPVPLVKQKGGQYAGFEISSHNDDFIIKIPFGRWQVRKEIDKYRPWEKFNFEQVRKSPKPISLLLSTQRRKRNKGWSKDEGTEAEIRKVMNGDYQTSYIEVKRGSKIGEKSAWMLCLSIDVPKIDKGVDPSIIGGIDVGVKSPLVCAINNVLSRYSISDNDLFHFNKKMFARRRILLKKNGHKRAGHGAKNKLKPITIMTEKSKRFRKKLIERWACEIADFFIKNKVGTVQMENLESMKRKEDSYFNIRLRGFWPYAEMQNKIEFKLKQYGIVVRKVAPNNTSKTCSQCGHLNNHFNFEYRKKNKFPYFKCEKCNFKENADYNAALNISNPQLKSTKGEP

SEQ ID NO: 2289 - protein, 726 aa, synthetic construct
SEVEFSHEYWMRHALTLAKRARDEREVPVGAVLVLNNRVIGEGWNRAIGLHDPTAHAEIMALRQGGLAMQNYRLIDATLYVTFEPCVMCAGAMIHSRIGRVVFGVRNNKHGAAGSLVNVLNYPGMNHRVEITEGILADECAALLCDFYRMPRQVFNARKKAQSSINSGGSSGGSSGRETPGTSGSATPESSGGSSGGSAKNTITKTLKLRIVRPYNSAEVEKIVADEKDNRERIALEKNKGKVKEACSKHLKVAAYCTTQVERNACLFCKARKLDDKFYQELRGQFPDAVFWQEIGEIFRQLQRQAAEIYNQSLIELYYEIFIKGKGFANASSAEHYLSDVCYTRAAELFKNAAIASGLRGKVKSNFRLKELKNMKSGLPTTKSDNFPIPLVKQKGGQYTGFEISSHNDDFVIKIPFGRWQVKREIDKYRPWERFDFEQVRKSPKPISLLLSTQRRKRNKGWSKDEGTEAEIRKVMNGDYQTSYIEVKRGSKIGEKSAWMLNLSIDVPKIDKGVDPSVIGGIDVGVKFPLVCAINNAFSRYSISDNDLFHFNKKMFARRRILLKKNRHKRAGHGAKNKLKPITIMTEKSKRFRKKLIERWACEIADFFIKNKVGTVQMENLESMKRKEDSYFNIRLRGFWPYAEMQNKIEFKLKQYGIEIRKVAPNNTSKTCSKCGHLSNYFNFEYRKKNKFPHFKCEKCNFKEDADYNAALNISNPKLKSTKEEP

SEQ ID NO: 2290 - protein, 726 aa, synthetic construct
SEVEFSHEYWMRRALTLAKRARDGREVPVGAVLVLNNRVIGEGWNRAIGLHDPTAHAEIMALRQGGLVMQNYRLIDATLYVTFEPCVMCAGAMVHSRIGRVVFGVRNGKRGAAGSLMNVLDYPGMGHRVEITEGILADECAALLCDFYCMPRQVFNAQKRAQSSINSGGSSGGSSGSETPGTSESATPKSSGGGSSGSAKNTITKTLQLRIVRPYNSAEVEKIVADEKNNREKIALEKNKDKVKEACSKHLKVASYCTTQVERNACPFCKARKLDDKFYQKLRGQFPDAVFWQELGEILRQLQKQAAEIYNQSLIELYYEIFIKGRGFANASSVEHYLSDVCYTRAAELFKNAAIASGLRGKVKSNFRLKELKNMKSGLPTTKSDNFPIPLVKQKGGQYTGFEISNHNSDFIIKIPFGRWQAKKEIDKYRPWEKFDFEQVRKSPKPISLLLSTQRRKKNRGWSKDEGTEAEIKKVMNGDYQTSYIEVKRGSKIGEKSAWMLNLSIDVPKIDKGVDPRTIGGIDVGVKSPLVCAINNVLSRYSISDNDLFHFNKKMFARRRILLKKNGHKRAGHGAKNKLKPISILTEKSKRFRKKLIERWACEIASFFIKNKVGTVQMENLESMKRKEDSYFNIRLRGFWPYAEMQNKIEFKLKQYGIEIRKVAPNNTSKTCSKCGHLNNYFNFEYRKKNKFPHFKCEKCNFKENADYNAALNISNPKLKSTKEEP

SEQ ID NO: 2291 - protein, 726 aa, synthetic construct
SEVEFSHEYWMRHALTLAKRARDEREVPVGAVLVLNNRAIGVGWNRAIGLHDPTAHAEIMALRQGGLVMQNYRLVDATLYVTFEPCIMCAGAMIHSRIGRVVFGVRNSKRGAAGSLMNVLNYPGMNHRVEITEGILAGECAALLCDFYRMPRQVFNAQKKAQSNINSGGSSGGSSGSETPGISESPIPESSGGSSGGSAKNTITKTLKLRIVRPYNSAEVEKIVADEKNNREKIALEKNKDKVKEACSKHLKVAAYCTTQVERNACLFCKARRLDDKFYQKLRGQFPDAVFWQEISEIFRQLQRQAAEIYNQSLVELYYEIFIKGKGFANASSVEHYLSDVCYTRAAELFKNAAIASGLRGKVKSNFRLKELKNMKSGLPTTKSDNFPIPLVKQKGGQYTGFEISSHNDDFIIKIPFGRWQVKKEIDKYRPWEKFDFEQVRKSPKPISLLLSTQRRKRNKGWSKDEGTEAEIRKVMSGDYQTSYIEVKRGSKTGEKSAWVLNLSIDVPKIDKGVDPSIIGGIDVGVKSPLVCAINNALSRYSISDNDLFHFNKKMFARRRILLKKNRHRRAGHGAKNKLKPISILTEKSERFRKKLIERWACEIADFFIKNKVGTVQMENLEGMKRREDSYFNIRLRGFWPYAEMQNKIEFKLRQYGIEVRKVAPNNTSRTCSKCGHLNNYFNFEYRKKNKFPHFKCEKCNFKEDADYNAALNISNPKLRSTKEEP

SEQ ID NO: 2292 - protein, 726 aa, synthetic construct
SEVEFSHEYWMRHALTLAKRARDEREVPVGAVLVLNNRVIGEGWNRAIGLHDPTAHAEIMALRQGGLVMQNYRLTDATLYVTFEPCVMCAGAMIHSRIGRVVFGVRNSKRGAAGSLMNVLNYPGMNHCVEITEGILMDECAALLCDFYRMPRQVLSAQKKAQSSISSGGPSGGSSCSETPGASESVTPKSSGGSSTGSTKNTITKTLKLRIVRPYNSAEVEKIVADEKNSREKIALEKNKDKVKEACSEHLKVAAYCTTQVERNACLFCKARKLDDRFYQKLRGQFPDAVFWQEIGEIFRQLQKQAAEIYNQSLIELYYEIFIKGKGFAIASSVEHYLSCVCYTRAAELFKNAAIASGLRGKVKSNFRLKELKNMKSGLPTTKSDNFPIPLVKQKGGQYTGFEISSHNDDFIIKIPFGRWQVKKEIDKYRPWEKFDFEQVRKSPKPISLLLSTQRRKRNKGWSKDEGTEAEIRKVMNGDYQTSYIEVKRGSKIGEKSAWMLNLSIDVPKIDKGVDPSIIGGIDVGVKSPLVCAINNAFSRYSISDNDLFRFNKKMFARRRILLKKNRRKRAGHGAKNKLKPITIMTGKSERFRKKLIERWACEIADFFIKNKAGTVQMENLESMKRKEDSYFNIRLRGFWPYAEMQNKIEFKLKQYGIEIRKVAPNNTSKTCSKCGHLNNYFNFEYRKKNKFPHFKCEKCNFKENADYNAALNISNPKLKSTKEEP

SEQ ID NO: 2293 - protein, 726 aa, synthetic construct
SEVEFSHEYWMRHALALAKRARDEREVPVGAVLVLNNRAIGEGWNRAIGLHDPTAHAEIMALRQGGLVMQNYRLTDATLYVTFEPCVMCAGAMIHSRIGRVVFGVRNSKRGAAGSLMNVLNYPGMNHCVEITEGILVDECAALLCDFYRMPRQVLNAQKKAQSSISSGGSSGGSSGSETPGASGSVIPRSSGGSSAGSTKDTITKTLKLRIVRPYNSAEVEKVVADEKNNREKIAMEKNKDKVKEACSKHLKVAAYCTTQVERNACLFCKARKLDDKFYQKLRGQFPDAVFWQETGEIFRQLQRQAAEIYNQSLIELYYEIFIKGKGFANASSVEHYLSDVCYTRAAELFKNAAIASGLRGKVKGNFRLKELKNMKSGLPTTKSDNFPIPLVKQKGGQYTGFEISSHNDDFIIKIPFGRWQVKKEIDKYRPWEKFDFEQVRKSPKPISLLLSTQRRKRNKGWSKDEGTEAEIRKVMNGDYQTSYIEVKRGSKVGEKSAWMLNLSIDVPKIDKGVDPSIIGGIDVGVKSPLVCAINNAFSRYSISDNDLFHYNKKMFARRRILLKKNRHKRAGHGAKNKLKPISILTEKSKRFRKKLIERWACEIADFFIKNKVGTVQIENLESMKRKEDSYFNTRLRGFWPYAEMQNKIEFKLKQYGIEIRKVAPNNTSKTCSKCGHLNSYFNFEYRKKNKFPHFKCEKCNFKENADYNAALNISNPKLRSTKEEP

SEQ ID NO: 2294 - protein, 726 aa, synthetic construct
SEVEFSHEYWMRHALTLAKRARDEREVPVGAVLVLNNRVIGEGWNRTTGLHDPTAHAEIMALRQGGLVMQNHRLVDATLYVTFEPCVMCAGAMIHSRIGRVVFGVRNSKRGAAGSLTNVLNYPGMNHRVEITEGILVDECAALLCDFYRMPRQVFNAQKKAQSAINSGSSSGGSSGSETPGTSESPTPESSGGSPGGSAKSTITKTLKLRIVRPYNSAEVEKIVADEKNNREKIALEKNKDKVKEACSKHLKVAAYCTTQVERNACLFCKARKLDDKFYQKLRGQFPDAVFWQETGEIFRQLQRQAAEIYNQSLIELYYEIFIKGKGFANASSVEHYLSDVCYTRAAELFKNAAIASGLRGKVKSNFRLKELKNMKSGLPTTKSDNFPIPLVKQKGGQYTGFEISSHNDDFIIKIPFGRWQVKKEIDKYRPWEKFDFEQVRKSPKPISLLLSTQRRKRNKGWSRDEGTEAEIRKVMNGDYQTSYIEVKRGSKIGEKSAWMLSLSIDVPKIDKGVDPSIIGGIDVGVKSPLVCAINNAFCRYSISDNDLFHFNKKMFARRRILLKKSKHKRAGHGAKNKLKPITILTEKSGRFRKKLIERWACEIADFFIKNKVGTVQMENLEGMKRKEDSYFNIRLRGFWPYAEMQNKIEFKLKQYGIEIRKVAPNNTSKTCSKCGHLNSYFNFEYRKKNKFPHFKCEKCNFKEDADYNAALNISNPKLKSTKEEP

SEQ ID NO: 2295 - protein, 726 aa, synthetic construct
SEVEFSHEYWMRHALTLARRARDEREVPVGAVLVLNNRVIGGGWNRTVGLHDPTAHAEIMALRQGGLVMQNYRLIDATLYVTFEPCVMCAGAMIHSRIGRVVFGVRNSKRGAAGSLMNVLNYPGMNHCVEITEGILVDECAALLCDFYRMPRQVLNAQKKAQSSINSGGSSSGSSGSETPSTCESATPESSGGSSGGSARNTITKTLQLRIVRPYNSAEVEKIVTDEKNAREKIALEKNKDKVKEACSEHLKVAAYCTTQVERSACLFCKARKLDDKFYQKLRGQFPDAVFWQEIGEIFRQLQKQAAEIYNQSLIELYYEIFIKGKGFANASSVEHYLSDVCYTRAAELFKNAAIASGLRGKVKSNFRLKELKNMKSGLPTTKSDNFPIPLVKQKGGQYTGFEISSHNDDFIIKIPFGRWQVKKEIDKYRPWEKFDFEQVRKSPKPISLLLSTRRRKRNKGWSKDEGTEAEIRKVMNGDYQTSYIEVKRGSKIGEKSAWMLNLSIDVPKIDKGVDPSTIGGIDVGVKSPLVCAINNAFCRYSIGDNDLFRFNKKMFARRRILLKKNRHQRAGHGAKNKLKPITILTEKSERFRKKLIERWACEIADFFVKNRVGTVQMENLESMKRKEDSYFNIRLRGFWPYAEMQNKIEFKLKQYGIKVRKVAPNNTSKTCSKCGHLNNYFSFEYRKKNKFPHFKCEKCNFKENADYNAALNISNPKLKSTKEEP

SEQ ID NO: 2296 - protein, 726 aa, synthetic construct; identical to SEQ ID NO: 684

SEQ ID NO: 2297 - protein, 725 aa, synthetic construct
SEDEFSHEYWMRHALTLAKRARDGREVPVGAVLVLNNRVIGEGWNRAIGLHDPTAHAEIMALRQGGLVMQNYRLIDATLYVTFEPCVMCAGAMIHSRIGRVVFGVRNNKHGAAGSLVNVLNYPGMNHRVEITEGILADECAALLCDFYRMPRQVFNARKKARSNINSGGSSGGSSGSETPGTSESATPESSGGSSGGSTKNTITKTLKLRIVRPYNSAEVEKIVADEKNNREIALEKNKDKVKEACSKHLKVAAYCTTQVERNACLFCRARRLDDKFYQKLRGQFPDAVFWQEIGEVFRQLQKQAAEIYNQSLVELYYEIFIKGKGIANASSVEHYLSDVCYTRAAELFKNAAIASGLRNKIKSNFRLKELRNMKSGLPTTRSDNFPIPLVRQKGGQYTGFEISSHNDDFIIKIPFGRWQAKKEIDKYRPWEKFDFEQVRKSPKPISLLLSTQRRKRNKGWSKDESTEAEIRKVMNGDYQTSYIEVKRGSKIGEKSAWMLNLSIDVPKIDKGVDPSIIGGIDVGVKSPLVCAINNAFSRYSISDNDLFHFNKKMFARRRILLKKNRHKRAGHGAKNKLKPISILTEKSKRFRKKLIERWACEIADFFIKNKVGTVQMENLESMKRKEDSYFNIRLRGFWPYAEMQNKIEFKLKQYGIEIRKVAPNNTSKTCSKCGHLNNYFNFEYRRENKFPHFKCEKCNFKEDADYNAALNISNPKLKSTKEEP

SEQ ID NO: 2298 - protein, 726 aa, synthetic construct
SEVEFSHEYWMRHALTLAKRARDEREVPVGAVLVLNNRVIGEGWNRAIGLHDPTAHAEIMALHQGGLVMQNYRLIDATLYVTFEPCVMCAGAMIHSRIGRVVFGARNSKRGAAGSLMNVLSYPGMNHRVEITEGVLADECAALLCDFYRMPRRVFNAQKKAQSSINSGGSSGGGSGSETPSTSESTTPESSGGSSGGPAKNTITKTLKLRIVRPYNSAEVEKIVADEKNNREKIALEKNRDKVKEACSKHLKVAAYCTTQVERNACLFCKARKLDDKFYQKLRGQFPDAVFWQELGEILRQLQKQAAEIYNQSLIELYYEIFIKGKGFANASSVEHYLSDVCYTRAAELFKNAAIASGLRGKVKSNFRLKELKNMKSGLPTTKSDNFPIPLVRQKGGQYTGFEISNHNDDFIIKIPFGRWQVKKEIDKYRPWEKFDFEQVRRSPKPISLLLSTQRRKRNKGWSKDEGTEAEIRKVMNGDYQTSYIEVKRGSKIGEKSAWMLNLSIDVPKIDKGVDPSIIGGIDVGVKSPLVCAINNAFSRYSISDNDLFHFNKKMFARRRILLKKSRHKRAGHGAKNKLKPITILTEKSRRFRKKLIERWACEIADFFIKNKVGTVQMENLESMKRKEDSYFNIRLRGFWPYAEMQDKIEFKLKQYGIKVRKVAPNNTSKTCSKCGHLNNYFSFEYRKKNKFPHFKCEKCNFKENADYNAALNISNPKLKNIKGEP

SEQ ID NO: 2299 - protein, 726 aa, synthetic construct
SEVEFSHEYWMRHALTLAKRARDEREVPVGAVLVLNNRVIGEGWNRAVGLHDPTAHAEIMALRQGGLVMQNYRLTDATLYVTFEPCVMCAGAMIHSRIGRVVFGVRNSKRGAAGSLMNVLNYPGMNHCVEITEGILVDECAALLCDFYRMPPQVLNARKKAQSSISSGGSSGGSNGSKTPGASESATPESSGGSSGGSAKNTITKTLKLRIVRPYNSAEVEKIVADEKNNREKIALEKNKNKVKEACSKHLKVAAYCTTQVERNACPFCRARKLDDKFYQKLGGQFPDAVFWQEIGEIFGQLQKQAAEIYNQSLIELYYEIFIKGKGFANSSSVEHYLSDVCYTRAAELFKNAAIASGLRGKVKSNFRLKELKNMKSGLPTTKSDNFPIPLVKQKGGQYTGFEISSHNDDFIIKIPFGKWQVKKEIDKYRPWEKFDFEQVRKSPKPISLLLSTQRRKRNKGWGKDEGTEAEIRKVMNGDYQTSYIEVKRGSKIGEKSAWMLSLSIDVPKIDKGVDPSIIGGIDVGVKSPLVCAINDAFSRYSISDNDLFRFNKKMFAMRRILLKKNRHKRAGHGAKNKLKPITILTEKSKRFRKKLIERWACEIADFFIKNKVGTVQMENLESMKRKEDSYFNIRLRGFWPYAEMQDKIEFKLKQYGIEIRKVAPNNTSKTCSRCGHLNNYFNFEYRRKNKFPHFKCEKCNFKENADYNAALNISNPKLKSTKEEP

SEQ ID NO: 2300 - protein, 726 aa, synthetic construct
SEVEFSHEYWMRHALTLAKRARDEREVPVGAVLVLNNRVIGEGWNRAIGLHDPTAHAEIMALRQGGLVMQNYRLVDATLYVTFEPCVLCAGAMVHSRIGRVVFGVRNSKRGAAGSLMNVLSYPGMNHRVEITEGILADECAALLCDFYRMPRRVFNAQKKARSNINSGGSSGGSSGSETPGTSESATPESSGGSSGGSAKNTITKTLKLRIVRPYNSAEVEKIVADEKNNREKVALERNKDKVKEACSKHLKVVAYCTTQVERNACLFCKARKLDDKFYQKLRGQFPDAVFWQEIGEIFRQLQKQAAEIYNQSLIELYYEIFIKGKGIASASRVGHYLSDVCYTRAAELFKNAAIASGLRSKIKSNFRLKELKNMKSGLPTTKSDNFPIPLVKQKGGQYTGFEISNHNSDFIIKIPFGRWQVKREIDKYRPWEKFDFEQVRKSPKPISLLLSTQGRRRNKGWSKDEGTEAEIKKVMNGDYQTSYIEVKRGSKIGEKSTWMLNLSIDVPKIDKGVDPSIVGGIDVGVKSPLVCAINNSFSRYSICDNDLFRFNKKMFARRRILLKKNRHKRAGHGAKNKLKPITILTKKSERFRKKLIERWVCEVADFFVKNKVGTVQMENLESMKRREDSYFNIRLRGFWPYAEMQNKIEFKLKQYGIKVRRVAPNNTSKTCSKCGHLNNYFSFEYRKKNKFPHFKCEKCNFKENADYNAALNISNPKLKSTKEEP

SEQ ID NO: 2301 - protein, 726 aa, synthetic construct
SEVEFSHEYWMRHALTLAKRARDEREVPVGAILVLNNRVIGEGWNRAIGLHDPTAHAEIMALRQGGLVMQNYRLTDATLYATFEPCVMCAGAMIHSRIGRVVFGVRNSKHGAAGSLMNVLNYPGMNHRVEITEGILADECAGLLCDFYRMPRQVFSARKKAQSSINPGGSSGGSSGGKAPGTSESATLESSGGSSGGSAKNSITKTLKLRIVRPYNSAEVEKIVADEKNNREKTALEKNKGKVKEACSKHLKVAAYCTTQVERNACLFCKARKLDDKFYQKLRGQFPDAVFWQEIGEIFRQLQKQAAEIYNQSLIELYYEIFIKGKGFANASSVEHYLSDVCYTRAAELFKNAAIASGLRGKVKSNFRLKELKNMKSGLPTTKSDNFPIPLVKQKGGQYTGFEISSHNDDFIIKIPFGRWQVKKEIDKYRPWEKFDFEQVRKSPKPISLLLSTQRRKRNRGWSKDEGTEAEIRKVMNGDYQTSYIEVKRGSKIGEKSAWVLNLSIDVPKIDKGVDPSIIGGIDVGVKSPLVCAINNAFSRYSISDNDLFHFNKKVFARRRILLKKNRHRRAGHGAKNKLKPITILSEKSKRFRKKLIERWACEIADFFIKNKVGTVQMENLESMKRKEDSYFNIRLRGFWPYAEMQNKIEFKLKQYGIETRKVAPNNTSRTCSKCGHLNNYFSFEYRKKNKFPHFKCEKCNFKEDADYNAALNISNPKLKSTKEEL

SEQ ID NO: 2302 - protein, 726 aa, synthetic construct; identical to SEQ ID NO: 684

SEQ ID NO: 2303 - protein, 726 aa, synthetic construct
GEVEFSHEYWMRRALTLAKRARDEREVPVGAILVLNNRVIGEGWNRAIGLHDPTAHAEITALRQGGLVMQNYRLIDATLYVTFEPCVMCAGAMIHSRIGRVVFGVRNSKHGAAGSLVNVLNYPGMNHRVEITEGILVDECAALLCDFYRMPRQVLNAQKKARSSISSGGSSGGSSGSETPGASESATPKSSGGSSAGSTKNTITKTLKLRIVRPYNSAEVEKIVTDEKNNREKIALEKNKDKVKEACSKHLKMASYCTTQVERNACLFCKARKLDDKFYQKLRGQFPDAVFWQELGEIFRQLQKQAAEIYNQSLIELYYEIFIKGKGFANASSVEHYLSDVCYTRAAELFKNAAIASGLRGKVKSNFRLKELKNMKSGLPTTKSDNFPIPLVKQKGGQYTGFEISSHNDDLIIKIPFGRWRVKKEIDKYRPWEKFDFEQVRKSPKPISLLLSTQRRKRNKGWSKDEGTEAEIRKVMNGDYQTSYIEVKRGSKIGEKSAWMLNLSIDVPKIDKGVDPSIIGGIDVGVKSPLVCAINNSFSRYSICDNDLFRFNKKMFARRRILLKRNRHKRAGHGAKNKLKPITILTEKSKRFRRKLIERWACEIADFFIKNKVGTVQMENLESMKRKEDSYFNIRLRGFWPYAEMQDKIEFKLKQYGIEIRKVAPNNTSKTCSRCGHLNNYFNFEYRRKNKFPHFKCEKCNFKENADYNAALNISNPKLRSTKEEP

SEQ ID NO: 2304 - protein, 726 aa, synthetic construct
GEVEFSHEYWMRHALTLAKRARDGREVPVGAVLVLNNRVIGEGWNRAIGLHDPTAHAEIMALRQGGLVMQNYRLIGATLYVTFEPCVMCAGAMVHSRIGRVVFGVRNSKRGAAGSLMNVLDYPGMDHRVEITEGILADECAALLCDFYRMPHQVFNAQKKAQSSINSGGSSGGSSGSVTPGPSESATQESFGGSSGGSAKNTITKTLKLRIVRPYNSAEVEKIVADEKNNREKIALEKNKDKVKEACSKHLKVAAYCTTQVERNACLFCKARKLDDKFYQKLRGQFPDAVFWQEISEIFRQLQKQAAVIYNQGLIELYYEIFIKGKGIANASRVEHYLSNVCYTRAAELFKNAAIASGLRNKIKSNFRLKELRNMKSGLPTTKSDNFPIPLVRQKGGQYTGFEISNHDGDFIIKIPFGRWRVKKEINKHRPWEKFDFEQVRKSPKPISLLLSTQRRKRNKGWSKDEGTEAEIRKVMNGDYQTSYIEVKRGSKIGEKSAWMLSLSIDVPKIDKGVDPSIIGGIDVGVKSPLVCAINNTFSRYSISDNDLFRFNKKMFARRRILLGKNRHKRAGHGVKNKLKPITILTEKSGRFRKKLIERWACEIADFFVKNKVGTVQMENLESMKRKEDSYFNIRLRGFWPYAEMQNKIEFKLKQYGIKVRKVAPSNTSKTCSKCGHLNNYFSFEYRKKNKFPHFKCEKCNFKENADYNAALNISNPKLKSTKEEP

SEQ ID NO: 2305 - protein, 726 aa, synthetic construct
SEVEFSHEYWMRHALTLAKRARDEREVPVGAVLVLNNRVIGEGWNRAIGLHDPTAHAEIMALRQGGLAMQNYRLIDATLYVTFEPCVMCAGAMIHSRIGRVVFGVRNSKHGAAGSLVNVLNYPGMNHRVEITEGILADECAALLCDFYRMPRQVFNARKRAQSSINPGGSSGGSSGSGTPGISESATPESSGGSSGGSAKNTITKTLKLRIVRPYNSAEVEKIVADEKNNREKIALEKNKDKVKEACSKHLKVAAYCTTQVERNACPFCKARKLDDRFYQKLRGQFPDAVFWQEIGEIFRQLQKQAAEIYNQSLIELYYEIFIKGKGLANASSVEHYLSGVCYTRAAELFKNAAIASGLRGKVKSNFKLKELKSMKSGLPTTKSDNFPIPLVKQKGGQYTGFEISSHNDDFIIKIPFGRWQVKKEIDRYRPWEKFDFEQVRKSPKPISLLLSTQRRKGNKGWSKDEGTEAEIRKVMNGDYQTSYIEVKRGSKIGEKSAWMLNLSIDVPKIDKGVDPSIIGGIDVGVKSPLVCAVNNAFSRYSISDNELFHFNKKMFARRRILLKKNRHKRAGHGAKNKLKPISILTEKSERFRKKLIEKWACEIADFFIKNKVGTVQMENLESMKRKEDSYFNIRLRGFWPYAEMQNKIEFKLKQYGIEIRKVAPNNTSKTCSKCGHLNSYFNFEYRKKNKFPHFRCEKCNFRENADYNAALNISNPKLRSTKEEP

SEQ ID NO: 2306 - protein, 726 aa, synthetic construct
NEVEFSHEYWMRHALTLAKRARDEREVPVGAVLVLNNRVIGEGWNRTTGLHDPTAHAEIMALRQGGLVMQNHRLVDATLYVTFEPCVMCAGAMIHSRIGRVVFGVRNSKRGAAGSLTNVLNYPGMNHRVEITEGILADECAALLCDFYRMPRQVFNARKKAQSSTNPGGSSGGSSGSETPGTSESPTPESSGGSSGGSAKNTITKTLKLRIVRPYNSAEVEKIVAEEKNNREKIALEKNKDKVKEACSKHLKVAAYCTTQVERNACLFCKARKLDDKFYQKLRGQFPDAVFWQELGEILRQLQKQAAEIYNQSLIELYYEIFIKGRGFANAGSVEHYLSDVCYTRAAELFKNAAIASGLRGKVKSNFRLKELKNMKSGLPTTKSDNFPIPLVKQKGGQYTGFEISSHNSDFIIKIPFGRWQVKEEIDKYRPWEKFDFEQVRKSPKPISLLLSTQRRKKNKGWSKDEGTEAEIRRVMNGDYQTSYIEVKRGSKIGEKSAWMLNLSIDVPKIDKGVDPSIIGGIDVGVKSPLVCAINNSSSRYSICDNDLFRFNKKMFARRRILLKKNRHKRAGHGAKNKLKPITILTKKSERFRKKLIERWVCEVADFFIKNKVGTVQMENLESMKRKEDSYFNIRLRGFWPYAEMQNRIELKLKQYGIEIRKVAPNNTSKTCSKCGHLNNYFNFEYRKKNKFPHFKCEKCNFKENADYNAALNISNPKLKSTKEEP

SEQ ID NO: 2307 - protein, 726 aa, synthetic construct
SEVEFSHEYWMRHALTLAKRARDEREVPVGAILVLNNRVIGEGWNRAIGLNDPTAHAEIMALRQGGLVMQNYRLIDATLYVTFEPCVMCAGAMIHSRIGRVVFGVRNNKHGAAGSLVNVLNYPGMNHRVEITEGILADECAALLCDFYRMPRQVFNARKKAQSSINPGGSSGGSGGSETPGTSESATPESSGGSSGSSAKNTITKTLKLRIVRPYNSAEVEKIVADEKNNREKIALEKNKDKVKEACSKHLKVAAYCTTQVERNACLFCKARRLDDKFYQKLRGQFPDAVFWQEIGEIFRQLQKQAAEIYNQSLVELYYEILIKGKGIANASSVEHYLSDVCYTRAAELFKNAAIASGLRNKIKSNFRLKELRNMRSGLPTAKSDNFPIPLVKQKGGQYTGFEISSHNDDFIIKIPFGRWQVKKEIDKYRPWEKFDFEQVRKSPKPISLLLSTRRRKRNKGWSKDEGTEAEIRKVMNGGYQTSYIEVKRGSKVGEKSAWMLNLSIDVPKIDKGADPSIIGGIDVGVKSPLVCAINNAFSRYSISDNDLYRFNKKMFARRRILLKKNRHKRAGHGAKNKLKPISVLTEKSERFRKKLIERWACEIADFFIKNKVGTVQMENLESMKRKEDSYFNIRLRGFWPYAEMQNKIEFKLKQYGIVVRKVAPNNTSKTCSKCGHLNNYFNFEYRKKNKFPHFKCEKCNFKEDADYNAALNISNPKLKNTKGEP

SEQ ID NO: 2308 - protein, 726 aa, synthetic construct
SEVGFSHEYWMRHALTLARRARDGREVPVGAVLVLNNRVIGEGWNRAIGLHDPTAHAEIMALRQGGLVMQNYRLIDATLYVTFEPCVMCAGAMIHSRVGRVVFGVRNNKHGAAGSLVNVLNYPGMNHRVEITEGILADECAALLCDFYRMPRQVFNARKKAQSGINPGGSSGGSSGSETPGTSESATPESSGGSSGGSAKNTITKTLKLRIVRPYNSAEVEKIVADEKNNREKTALEKNKDKVKEACSKHLKVAAYCTTQVERNACLFCKARKLDDKFYQKLRGQFPDAVFWQEVGEIFRQLQKQAAEIYNQSLIELYYEIFIKGKGFANASSVEHYLSDVCYTRAAELFKNAAIASGLRGKVKSNFRLKELKNMKSGLPTTKSDNFPIPLVKQKGGRYTGFEISSHNDDFIIKIPFGRWQGKKEVDKYRPWEKFDFEQVRKSPKPISLLLSTQRRKRNKGWSKDEGTEAEIKKVMNGDYQTSYIEVKRGSRIGEKSAWMLSLSIDVPKIDRGVDPSIIGGIDVGVKSPLVCAINNASSRLSISDNDLFRFNKKMFARRRILLKKNGHKRAGHGAKNKLKPITILTEKSVRFRKKLIERWACEIADFFIRNKVGTVQMENLEGMKRKEDSYFNIRLRGFWPYAEMQNKIEFKLKQYGIEIRKVAPNNTSKTCSKCGHLNNYFSFEYRKKNKFPHFKCEKCNFKENADYNAALNISNPKLKSTKEEP

SEQ ID NO: 2309 - protein, 726 aa, synthetic construct
SEVEFSHEYWMRHALTLAKRARDEREVPVGAVLVLNNRVIGEGWNRAIGLHDPTAHAEIMALRQGGLVMQNYRLTDATLYVTFEPCVMCAGAMIHGRIGRVVFGARNSKRGAAGSLMNVLNYPGMNHCVEITEGILVDECAALLCDFYHMPRQVLNAQKKAQSSISSGGSSGGSSGSETPGASESVTPKSSGGSSAGSTKNTITKTLKLRIVRPYNSAEVEKIVADEKNSREKIALEKNKDKVKEACSEHLKVAAYCTTQVERNACLFCKARKLDDRFYQKLRGQFPDAVFWQEIGEIFRQLQKQAAETYNQSLIELYYEIFIKGKGFANASSVEHYLSDVCYTRAAELFKNAAIASGLRGKVKSNFRLKELKNMKSGLPTTKSDNFPIPLVKQKGGQYTGFEISSHNNDFIIKIPFGRWQVKEEIDKYRPWEKFDFEQVRKSPKPISLLLSTQRRKRNKGWSKDEGTEAEIRKVMNGDYQTSYIEVKRGSKIGEKSAWMLNLSIDVPKIDKGVDPSIIGGIDVGVKSPLVCAINNAFIRYSISDNDLFHFNKKMFARRRILLKKNRHKRAGHGAKNKLKPISILTEKSKRFRKKLIERWACEIADFFIKNKVGTVQMENLESMKRKEDSYFNIRLRGFWPYAEMQNKIEFKLKQYGIEIRKVAPNNTSKTCAKCGHLNNYFNFEFRKKNKFPHFKCEKCNFKENADYNAALNISNPKLKSTKEEP

SEQ ID NO: 2310 - protein, 726 aa, synthetic construct; identical to SEQ ID NO: 684

SEQ ID NO: 2311 - protein, 726 aa, synthetic construct
SEVEFSHEYWMRHALTLAKRARDEREVPVGAVLVLNNRVIGEGWNRAIGLHDPTAHAEIMALRQGGLVLQNYRLVDATLYVTFEPCVLCAGAMVHSRIGRVVFGARNSKRGAAGSLMNILNYPGMNHRVEITEGILADECAALLCDFYRMPRQVFNAQKKAQSSINSGGSSSGSSGSETPSASESATPESSGGSSGGSARNTITKTLQLRIVRPYNSAEVEKIVTDEKNNREKIALEKNKDKVKEACSKHLKMASYCTTQVERNACLFCKARKLDDKFYQKLRGQFPDAVFWQELGGIFRQLQKQAAEIYNQSLIELYYEIFIKGKGITNASRVEHYLSDVCYTRAAELFKNAAIASGLRSKVRSNFRLKELKNMKSGLPTTKSDNFPIPLVKQKGGQYTGFEISSHNDDFIIKIPFGRWQVKKEIDKYRPWEKFDFERVRKSPKPISLLLSTRRRKRNKGWSKDEGTEAEIKRVMNGDYQISYIEVKRGSKIGEKSAWMLSLSVDVPKIDKGVDPSIIGGIDVGVKSPLVCAINNALSRYSISDNDLFHFNKKMFARRRILLRNNRHKRAGHGAKSKLKPITILTEKGERFRKKLIERWACEIANFFIKNKVGTVQMENLESMKRKEDSYFNVRLRGFWPYAEMQNKIEFKLKQYGIEIRRVAPNNTSRTCSKCGHLNNYFNFEYRKKNKFPHFKCEKCNFKENADYNAALNISNPKLKSTKEEP

SEQ ID NO: 2312 - protein, 726 aa, synthetic construct
SEVEFSHEYWMRHALTLAKRARDEREVPVGAVLVLNNRVIGEGWNRAIGLHDPTAHAEIMALRQGGLVLQNYRLIDATLYVTFEPCVMCAGAMIHSRIGRVVFGVRNSKHGAAGSLVNVLNYPGMNHRVEITEGILADECAALLCDFYRMPRQVFNARKRAQSSINSGGSSGGSSGSETPGTSESATPESSGGGSSGSAKNTITKTLQLRIVRPYNSAEVEKIVADEKNNREKIALEKNKDKVKEACSKHLKVAAYCTTQVERNACLFCKARKLDDKFYQKLRGQFPDAVFWQEIGEIFRQLQKQAAEIYNQSLIELYYEIFIKGKGFVNASSVEHYLSDVCYTRAAELFKNAAIASGLRNKIKSNFRLKELRNMKSGLPTTKSDNFPIPLVRQKGGQYTGFEISNHDGDFIIKIPFGRWQVKKEINKHRPWEKFDFEQVRKSPKPISLLLSTQRRKRNKGWSKDEGTEAEIRKVMNGDYQTSYIEVKRGSKIGEKSAWMLNLSIDVPKIDKGVDPSIIGGIDVGVKSPLVCAISNVLSRYSISDNDLFHFNKKMFARRRILLKKNGHKRAGHGAKNKLKPITIMTEKSKRFRKKLIERWACEIADFFIKNKVGTVQMENLESMKRKEDSYFNIRLRGFWPYAEMQNKIEFKLKQYGIVVRKVAPNNTSKTCSKCGHLNNYFDFEYRKKNKFPHFKCEKCNFKEDADYNAALNISNPKLKSSKGEP

SEQ ID NO: 2313 - protein, 726 aa, synthetic construct
SEVEFSHEYWMRHALTLAKRARDEREVPVGAILVLNNRVIGEGWNRAIGLHDPTAHAEIMALRQGGLVMQNYRLIDATLYVTFEPCVMCAGAMIHSRIGRVVFGVRNSKHGAAGSLVNVLNYPGMNHRVEITEGILADECAALLCDFYRMPRQVFNARKKAQSSINSGGSSGGSSGSETPGTSESATPESSGGGSSGSAKNTITKTLQLRIVRPYNSAEVEKIVADEKNNREKIALEKNKDKVKEACSKHLKVASYCTTQVERNACLFCKARKLDDKFYQKLRGQFPDAVFWQELGEIFRQLQKQAAEIYNQSLIELYYEIFIKGKGLANASSVEHYLSDVCYTRAAELFKNAAIASGLRGKVKSNFKLKELKSMKSGLPSTKSDNFPIPLVKQRGGQYTGFEISSHNDDFIIKIPFGRWQAKKEIDKYRPWEKFDLEQVRKSPKPISLLLSTQRRKRNKGWSKDEGTEAEIRKVMNGDYQTSYIEVKRGSKIGEKSAWMLSLSIDVPKIDKGVDPSIIGGIDVGVKSPLVCAINNAFCRYSISDNDLFHFNKKMFARRRILLKKSRHKRAGHGAKNKLKPISILTEKSKRFRKKLIERWACEIADFFIKNKVGTVQMENLESMKRKEDSYFNVRLRGFWPYAEMQNKIEFKLKQYGIEIRKVAPNNTSKTCSRCGHLNNYFSFEYRKKNKFPHFKCEKCDFKENADYNAALNISNPKLKGAKEEP

SEQ ID NO: 2314 - protein, 726 aa, synthetic construct
SEVEFSHEYWMRHALTLAKRARDEREVPVGAVLVLNNRVIGEGWNRAIGLHDPTAHAEIMALRQGGLVMQNYRLVDATLYVTFEPCVLCAGAMIHSRIGRVVFGVRNSKRGAAGSLMNVLNYPGMNHRVEITEGILADECAALLCDFYRMPRQVLSAQKKAQSSVSSGGSSGGSSGSETPGASGSVTPKSSVGSSAGSTKNTITKTLKLRIVRPYNSAEVEKIVADEKNNREKIALEKNKGKVKEACSKHLKVASYCTTQVERNACPFCKARKLDDKFYQKLRGQFPDAVFWQELGGILRQLQKQAAEIYNQSLIELYYEIFIKGRGFANASSVEHYLSDVCYTRAAELFKNAAIASGLRGKVKSSFRLKELKNMKSGLPTTKSDNFPIPLVKQKGGQYTGFEISSHNDDFIIKIPFGRWQVKKEIDKYRPWEKFDFEQVRKSPKPISLLLSTQRRKRNKGWSKDEGTEAEIKRVMNGDYQISYIEVKRGSKIGEKSAWMLSLSVDVPKIDKGVDPSIIGGIDVGVKSPLVCAINNALSRYSISDNDLFHFNKKMFARRRILLRNNRHKRAGHGAKSKLKPITILTEKGERFRKKLIERWACEIANFFIKNKVGTVQMENLESMKRKEDSYFNIRLRGFWPYAEMQNRIELKLKQYGIEIRRVAPNNTSRTCSKCGHLNNYFNFEYRKTNKFPHFKCEKCNFKENADYNAALNISNPKLKSTKEEP

SEQ ID NO: 2315 - protein, 726 aa, synthetic construct
SEVEFSHEYWMRRALTLAKRARDEREVPVGAVLVLNNRVIGEGWNRAIGLHDPTAHAEVMALRQGGLVMQNYRLTDATLYVTFEPCVMCAGAMIHSRIGRVVFGVRNSKRGAAGSLMNVLNYPGMNHCVEITEGILAGECAALLCDFYRMPRRVLNAQKKAQSNINSGGPSGGSSGSETPGTSESPTSEGSSGSSGGSARNAITKTLKLRIVRPYNSAEVEKIVADEKNNREKIALEKNKDKVKEACSKHLKVAAYCTTQVERNACLFCKARKLDDKFYQKLRGQFPDAVFWQELGEIFRQLQKQAAEIYNQSLIELYYEIFIKGKGFANASSVEHYLSGVCYTRAAELFKNAAIASGLRGKVKSNFRLKELKNMRSGLPTTRSDNFPIPLVKQKGGQYTGFEISSHNDDFIIKIPFGRWQVKKEIDKYRPWEKFDFEQVRKSPKPISLLLSTRRRKRNKGWSKDEGTEAEIRKVMNGDYQTSYIEVKRGSKTGEKSAWMLNLSIDVPKIDKGVDPSIIGGIDVGVKSPLVCAINNAFSRYSISDNDLFRFNKKMFARRRILLRKNRHKRAGHGARNKLKPISILTGKSERFRKKLIERWACEIADFFIKNKAGTVQMENLESMKRKEDSYFNIRLRGFWPYAEMQNKIEFKLKQYGIEIRKVAPNNTSKICSKCGHLNNYFNFEYRKKNKFPHFKCEKCNFKENADYNAALNISNPKLKSTKEEP

SEQ ID NO: 2316 - protein, 726 aa, synthetic construct
SEVEFSHEYWMRHALTLAKRARDEREVPVGAVLVLNNRVIGEGWNRAIGLHDPTAHAEIMALRQGGLAMQNYRLVDATLYVTFEPCVLCAGAMVHSRIGRVVFGVRNSKRGAAGSLMNVLNHPGMNHRVEITGGILADECAALLCDFYRMPRQVFNAQKKARSNINPGGSSGGSSGSETLGTSESATPKSSGGSSAGSTKNTITKTLKLRIVRPYNSAEVEKIVADEKNSREKIALERNKDKVKEACSEHLKVAAYCTTQVERSACLFCKARKLDDGFYQKLRGQFPDAVFWQETGEIFRQLQRQAAEIYNRSLIELYYEIFIKGKGFANASSVEHYLSDVCYTRAAELFKNAAIASGLRGKVKSNFRLKELKNMKSGLPTTKSDNFPIPLVKQKGGQYTGFEISSHDGDFIIKIPFGRWQMKKEINKHRPWEKFDFEQVRKSPKPISLLLSTQRRKRNKGWSKDEGTEAEIRKVMNGDYQTSYIEVKRGSKIGEKSAWMLNLSIDVPKIDKGVDPSIIGGIDVGVKSPLVCAINNAFSRYSISDNDLFHFNKKVFARRRILLKKNRHRRAGHGAKNKLKPITILTEKSKRFRKKLIERWACEIADFFIKNKVGTVQMENLESMKRKEDSYFNIRLRGFWPYAEMQNKIEFKLKQYGIKIRKVAPNNTSRTCSECGHLNNYFSFEYRKKNKFPHFKCEKCNFKEDADYNAALNISNPKLKSTKEEP

SEQ ID NO: 2317 - protein, 726 aa, synthetic construct
SEVELSHEYWMRHALTLAKRARDEREVPVGAILVLNNRVIGEGWNRAIGLHDPTAHAEIMALRQGGLVLQNYRLVDATLYVTFEPCVLCAGAMVHSRIGRVVFGARNSKRGAAGSLMNILNYPGMNHRVEITGGVLADECAALLCDFYRMPRQVFNAQKKAQSSINSGGSSGGSSGSGTPGTSESPTPESSGGSPGGSAKNTITKTLKLRIVRPYNSAEVEKIVADEKNNREKIALEKNKDKVKEACSKHLKVAAYCTTQVERNACLFCKARKLDDKFYQKLRGQFPDAVFWQELGEIFRQLQKQAAEIYNQSLIELYYEIFIKGKGFANASSVEHYLSDVCYTRAAELFKNAAIASGLRGKVKSNFRLKELKNMKSGLPTTKSDNFPIPLVKQKGGQYTGFEISNHNDDFIIKIPFGRWQVKKEIDKYRPWEKFDFEQVRKSPKPISLLLSTQRRKRNKGWSKDEGTEAEIRKVMNGDYQTSYIEVKRGSRTGEKSAWMLNLSIDVPKIDKGVDPSIIGGIDVGVKSPLVCAINNAFSRYSISDNDLFRFNKKMFARRRILLKKNRHKRAGHGAKNKLKPISILTGKSERFRKKLIERWACEIADFFTKNKVGTVQMENLESMKRKEDSYFNIRLRGFWPYAEMQNKIEFKLKQYGIEIRKVAPNNTSKTCSKCGHLNNYFNFEYRKKNKFPHFKCEKCNFKENADYNAALNISNPKLKSTKEEP

SEQ ID NO: 2318 - protein, 726 aa, synthetic construct
SVDEFSHEYWMRHALTLAKRARDGREVPVGAVLVLNNRVIGEGWNRAIGLHDPTAHAEIMALRQGGLVMQNYRLIDATLYVTFEPCVMCAGAMIHSRIGRVVFGVRNSKHGAAGSLVNVLNYPGMNHRVEITEGILADECAALLCDFYRMPRQVFNARKKAQSSINPSGSSGGSSGSVTPGTSESATPESSGGGFGGSAKNTITKTLQLRIVRPYNSAEVEKIVADEKNNREKIALEKNKDKVKEACSKHLKVASYCTTQVERNACLFCKARKLDDKFYQKLRGQFPDAVFWQELGEIFRQLQKQAAEIYNQSLIELYYEIFIKGKGLANASSVEHYLSDVCYTRAAELFKNAAIASGLRGKVKSNFKLKELKSMKSGLPSTKSDNFPIPLVKQRGGQYTGFEISSHNDDFIIKIPFGRWQAKKEIDKYRPWEKFDFEQVRKSPKPISLLLSTQRRKRNRGWSKDEGTEAEIRKVMNGDYQTSYIEVKRGSKIGEKSAWMLNLSIDVPKIDKGVDPSIIGGIDVGVKSPLVCAINNAFSRYSISDNDLFRFNKKMFARRRILLGKNRHKRAGHGVKNKLKPITILTEKSGRFRKKLIERWACEIADFFVKNKVGTVQMENLESMKRKEDSYFNIRLRGFWPYAEMQNKIEFKLKQYGIKVRKVAPNNTSKTCSKCGHLNNYFSFEYRKKNKFPHFKCEKCNFKENADYNAALNISNPKLKSTKEEP

SEQ ID NO: 2319 - protein, 726 aa, synthetic construct
SEVEFSHEYWMRHALTLAKRARDEREVPVGAILVLNNRVIGEGWNRAIGLHDPTAHAEIMALRQGGLVMQNYRLTDATLYVTFEPCVMCAGAMIHSRIGRVVFGVRNSKRGAAGSLMNVLNYPGMNHCVEITEGILVDECAALLCDFYRMPRQVLNAQKKAQSSISSGGSSGGSSGSETPGASGSVTPKSSGGSSAGSTKDTITKTLKLRIVRPYNSAEVEKVVADEKNNREKIAMEKNKDKVKEACSKHLKVASYCTTQVERNACLFCKARKLDDKFYQKLRGQFPDAVFWQELGGIFRQLQKQAAEIYNQSLIELYYEIFIKGKGLANASSVEHYLSDVCYTRAAELFKNAAIASGLRGKVKSNFRLKELKNMKSGLPTTKSDNFPIPLVKQKGGQYTGFEISSHNDDFIIKIPFGRWQVKKEIDKYRPWEKFDFEQVRKSPKPISLLLSTQRRKRNKGWSKDEGTEAEIRKVMNGDYQTSYIEVKRGSKTGEKSAWMLNLSIDVPKIDKGVDPSIIGGIDVGVKSPLVCAINNALGRFSISDNDLFHFNKKMFARRRILLRKNRHKRAGHGAKNKLKPISILTENSKRFRKKLIERWACEIADFFVKNKVGTVQMEDLESMKRRGDSYFNIRLRGLWPYAEMQNKIEFKLKQYGIEIRKVAPNNTSKTCSKCGHLNNYFNFEYRKKNKFPHFKCEKCNFKENADYNAALNISNPKLKNTKEEP

SEQ ID NO: 2320 - protein, 726 aa, synthetic construct
SEVEFSHEYWMRHALTLAKRARDEREVPVGAILVLNNRVIGEGWNRAVGLHDPTAHAEIMALRQGGLVMQNYRLIDATLYVTFEPCVMCAGAMIHSRVGRVVFGVRNSKHGAAGSLMNVLNYPGMNHRVEITEGILADECAALLCDFYRMPRRVFNARKKAQSSISSGGSSGGSSCSETPGASESVTPKSSGGSSAGSTKNTITKTLKLRIVRPYNSAEVEKIVADEKNSREKIALEKNRDKVKEACSEHLKVAAYCTTQVERNACLFCKARRLDDKFYQKLRGQFPDAVFWQEIGEIFRQLQKQAAEIYNQSLIELYYEIFIKGKGIANASSVEHYLSDVCYTRAAELFKNAAIASGLRNKVKSNFRLKELRSMKSGLPTTKSDNFPVPLVRQKGGQYTGFEISNHNSDFIIKIPFGRWQAKKEIDKYRPWEKFDFEQVRKSPKPISLLLSTQRRKRNKGWSKDEGTEAEIRKVMNGGYQTSYIEVKRGSKTGEKSAWMLNLSIDVPKIDKGVDPSNIGGIDVGVKSPLVCAINNAFSRYSISDNDLFHFNKKMFARRRILLKKNRHKRAGHGAKNKLKPISTLTERSKRFRKKLIERWACEIADFFIKNKVGTVQMENLESMKRKEDSYFNIRLRGFWPYAEMQNKIEFKLKQYGIEIRKVAPNNTSKTCSKCGHLNNYFNFEYRKKNKFPHFKCEKCNFKENADYNAALNISNPKLKSTKKEP

SEQ ID NO: 2321 - protein, 726 aa, synthetic construct
SEVEFSHEYWMRRALTLAKRARDEREVPVGAVLVLNNRVIGEGWNRAIGLHDPTAHAEIMALRQGGLVMQNYRLTDATLYVTFEPCVMCAGAMIHSRIGRVVFGVRNNKHGAAGSLVNVLNYPGMNHRVEITEGILADECAALLCDFYRMPRQVFNARKKAQSSINPGGSSGGSSGSETPGTSESATPESSGGSSGGSAKNTITKTLKLRIVRPYNSAEVEKIVADEKNNREKIALEKNKDKVKEACSKHLKVASYCTTQVERNACPFCKARKLDDKFYQKLRGQFPDAVFWQELGEILRQLQKQAAEIYNQSLIELYYEIFIKGEGFANASSVEHYLSDVCYTRAAELFKNAAIASGLRSKVRSNFRLKELKNMKSGLPTTKSDNFPIPLVKQKGGQYTGFEISSHNSDFIIKIPFGRWQEKEEIDKYRPWEKFDFEQVRRSPKPISLLLSTQRRKRNKGWSKDEGTEAEIRKVMNGDYQTSYIEVKRGSKIGEKSAWMLNLSIDVPRIDKGVDPSIIGGIDVGVKSPLVCAINNAFSRYSISDNDLFHFNKKMFARRRILLRKNRHKRAGHGARNKLKPITIMTEKSKRFRKKLIERWACEIADFFIKNKVGTVQMENLGSMKRKEDSYFNIRLRGFWPYAEMQNKIEFKLKQYGIEIRKVAPDNTSKTCSKCGHLNNYFNFEYRRKNKFPHFKCEKCNFKENADYNAALNISNPKLKSTKEEP

SEQ ID NO: 2322 - protein, 726 aa, synthetic construct; identical to SEQ ID NO: 684

SEQ ID NO: 2323 - protein, 726 aa, synthetic construct
SEVEFSHEYWMRHALTLAKRARDEREVPVGAILVLNNRVIGVGWNRAIGLHDPTAHAEIMALRQGGLVMQNYRLIDATLYVTFEPCVMCAGAMIHSRIGRVVFGVSNSKHGAAGSLVNVLNYPGMNHRVEVTEGILADECAALLCDFYRMPRQVFNARKKAQSSINSGGSSGGSSGSETPGTSESATPKSSGGSSGGSAKNTITKALKLRIVRPYNSAEVEKIVADEKNNRERIALEKNKDKVKEACSKHLKVAAYCTTQVERNACLFCKARKLDDKFYQKLRGQFPDAVFWQEIGEIFRQLQKQAAEIYNQSLIELYYEIFIKGKGFANASSVEHYLSDVCYTRAAELFKNAAIASGLRGKVKSNFRLKELKNMKSGLPTTKSDNFPIPLVKQKGGQYTGFEISSHNDDFIIKIPFGRWQVKKEIDRYRPWEKFDFEQVRKSPKPISLLLSTQRRKRNKGWSKDEGTEAEIRKVMNGDYQTSYIEVKRGSKTGEKSAWMLNLSIDVPKIDKGVDPSIIGGIDVGVKSPLVCAINNAFSRYSISDNDLFRFNKKMFARRRILLGKNRHKRAGHGAKNKLKPISILTGKSERFRKKLIERWACEIADFFIKNKVGTVQMENLESMKRKEDSYFNIRLRGFWPYAEMQNKIEFKLKQYGIGIRKVAPNNTSKTCSKCGHLNNYFNFEYRKKNKFPHFKCEKCNFKENADYNAALNISNPKLKSTKEEP

SEQ ID NO: 2324 - protein, 726 aa, synthetic construct; identical to SEQ ID NO: 684

SEQ ID NO: 2325 - protein, 726 aa, synthetic construct
SEVEFSHEYWMRHALTLAKRARDEREVPVGAVLVLNNRVIGVGWNRAIGLHDPTAHAEIMALRQGGLVMQNYRLTDATLYVTFEPCVMCAGAMVHSRIGRVVFGVRNSKRGAAGSLMNVLNYPGMSHCVEITEGILADECAALLCDYYRMPRQVFNARKKAQSSINSGGSSDGGSGSETPGTSESATPESSGGSSGGSAKNTITKTLKLRIVRPYNSAEVEKIVADEKNNREKIALEKNKDKVKEACSKHLKVAAYCTTQVERNACLFCKARRLDDKFYQKLRGRFPDAVFWQEIGEIFRQLQKQAAEIYNQSLIELYYEIFIKGKGFANASSVEHYLSDVCYTRAAELFKNAAIASGLRGKVKSNFRLRELKNMKSGLPTTKSDNFPIPLVKQKGGQYTGFEISNHNSDFIIKIPFGRWQVKKEIDKYRPWEKFDFEQVRKSPKPISLLLSTQRRKRNKGWSKDEGTEAEIRKVMNGDYQTSYIEVKRGSKIGEKSAWMLNLSIDVPKIDKGVDPSIIGGIDVGVKSPLVCAINNAFSRYSISDNDLFHFNKKMFARRRILLKKNRHKRAGHGAKNKLKPLTILTGKSKRFRKKLIERWACEIADFFIKNKVGTVQMENLESMKRKEDSYFNTRLRGFWPYAEMQNKIEFKLKQYGIEIRKVAPNNTSKTCSKCGHLNNYFNFEYRKRNKFPRFKCEKCNFKENADYNAALNISNPKLKSPKEEP

SEQ ID NO: 2326 - protein, 726 aa, synthetic construct
SEVEFSHEYWMRHALTLAKRARDEREVPVGAVLVLNNRVIGVGWNRAIGLHDPTAHAEIMALRQGGLVLQNYRLVDATLYVTFEPCVLCAGAMVHSRIGRVVFGARNSKRGAAGSLMNILNYPGMNHRVEITEGILADECAALLCDFYRMPRQVFNAQKKAQSSINSGGSSGGSSGSETPSTSESATPESSGGSSGGSAKNTITKTLQLRIVRPYNSAEVEKIVTDEKNNREKIALEKNKDKVKEACSKHLKMASYCTTQVERNACLFCKARKLDDKFYQKLRGQFPDAVFWQELGGIFRQLQKQAAEIYNQSLIELYYEIFIKGKGITNASRVEHYLSDVCYTRAAELFKNAAIASGLRGKVKSNFRLKELKNMKSGLPTTKSDNFPIPLVKQKGGQYTGFEISNHDGDFIIKIPFGRWQVKKEINKHRPWEKFDFEQVRKSPKPISLLLSTQRRKRNKGWSKDEGTEAEIRKVMNGDYQTSYIEVKRGSKIGEKSAWMLNLSIDVPKIDKGVDPSIIGGIDVGVKSPLVCAINNAFSRYSISDNDLFHFNKKMFARRRILLKKCKHKRAGHGAKNKLKPITILTEKSKRFRKKLIERWACEIADFFIKNKVGTVQMENLESMKKKEDSYFNIRLRGFWPYAEMQNKIEFKLKQYGIEIRKVAPNNTSRTCSKCGHLNNYFSFEYRKKNKFPHFKCEKCNFKEDADYNAALNISNPKLKGTKEEL

SEQ ID NO: 2327 - protein, 726 aa, synthetic construct
SEVEFSHEYWMRHALTLAKRARDEREVPVGAILVLNNRVIGEGWNRTTGLHDPTAHAEIMALRQGGLVMRNYRLTDATLYVTFEPCVMCAGAMIHSRIGRVVFGVRNSKRGAAGSLMNVLNYPGMNHCVEITEGILVDECAALLCDFYRMPRQVLNAQKKAQSSINPGGSSGGSSGSKTPGTSESATPESSGSGSSGSAKNTITKTLQLRIVRPYNSAEVEKIVADEKNNREKIALEKNKDKVKEACSKHLKVAAYCTTQVERNACLFCKARKLDDRFYQKLRGQFPDAVFWQEISEIFRQLQKQAAEIYNQSLIELYYEIFIKGRGFANAGSVEHYLSDVCYTRAAELFKNAAIASGLRGKVKSNFRLKELKNMKSGLPTTKSDNFPIPLVKQKGGQYTGFEIGSHNDDFIIKIPFGRWQVKKEIDKYRPWEKFDFEQVRKSPKPISLLLSTQRRRRNKGWSKDEGTEAEIRKVMNGDYQTSYIEVKRGSKIGEKSAWVLNLSIDVPKIDKGVDPSIIGGIDVGVKSPLVCAINNASSRYSISDNDLFRFNKKMFARRRILLKKNRHKRAGHGAKNKLKPISILTGKSERFRKKLIERWACEIADFFIKNKVGTVQMENLESMKKKEDSYFNIRLRGFWPYAEMQNRIEFKLKQYGIEIRKVAPNNTSKTCSKCGHLNNYFNFEYRKKNKFPHFKCEKCNFKENADYNAALNISNPKLKSTKEEP

SEQ ID NO: 2328 - protein, 726 aa, synthetic construct
SEVEFSHEYWMRHALALAKRARDEREVPVGAVLVLNNRVIGEGWNRAIGLHDPTAHAEIMALRQGGLVMQNYRLIDATLYVTFEPCVMCAGAMIHSRIGRVVFGVRNNKRGAAGSLMNVLNYPGMNHRVEITEGILADECAALLCDFYCMPRQVLNAQKKARSCINSGGSSGGSSGSETPGTSKSATPESSGGSSGGSAKNTITKTLKLRIVRPYNSAEVEKIVADEKDNRERIALEKNKDKVKEACSKHLKVAAYCTTQVERNACLFCKARRLDDKFYQKLRGQFPDAVFWQEIGEIFRQLQKQAAEVYNQSLVELYYEILIKGKGIANASSVEHYLSDVCYTRAAELFKNAAIASGLRNKIKSNFRLKELRNMKSGLPTTKSDNFPIPLVRQKGGQYTGFEISSHNDDFIIKIPFGRWQVKKEIDKYRPWERFDFEQVRKSPKPISLLLSTQRRKRNKGWGKDEGTEAEIRKVMNGDYQISYIEVKRGSKIGERSAWMLNLSIDVPKIDKGVDPSTIGGIDVGVKSPLVCAINNAFSRYSISDNDLFHFNKKMFARRRILLKKNRHRRAGHGARNKLKPITVLTEKSERFRKKLIERWACEIANFFIKNKVGTVQMENLESMKRREDSYFNIRLRGFWPYAEMQNKIEFKLKQYGIEIRKVAPNNTSKTCSKCGHLNNYFNFEFRKKNKFPHFKCEKCNFKENADYNAALNISNPKLKSTREEP

SEQ ID NO: 2329 - protein, 726 aa, synthetic construct
SEVEFSHEYWMRRALTLAKRARDEREVPVGAVLVLNNRVIGVGWNRAVGLHDPTAHAEIMALRQGGLVMQNYRLIEATLYVTFEPCIMCAGAMIHSRIGRVVFGVRNSKRGAAGSLMNVLNYPGMNHRVEVTEGILADECAALLCDYYRMPRQVFNARKKAQSSTNSGGSSDGGSGSETPGTSESATPESSGGSSGGSAKNTITKTLKLRIVRPYNSAEVEKIVADEKDSREKIALEKNKDKVTEACSEHLKVAAYCTTQVERNACLFCKARKLDDGFYQKLRGQFPDAVFWQEVGEIFRQLQKQAAEIYNQSLIELYYEIFIKGKGFANASSVEHYLSDVCYTRAAELFKNAAIASGLRGKVKSNFRLKELKNMKSGLPTTKSDNFPIPLVKQKGGQYTGFEISSHNSDFIIKIPFGRWQVKEEIDKYRPWEKFDFEQVRKSPKPISLLLSTQRRKKNKGWSKDEGTEAEIRRVMNGDYQTSYIEVKRGSKIGEKSAWMLNLSIDVPKIDKGVDPSIIGGIDVGVKSPLVCAINNSSSRYSICDNDLFRFNKKMFARRRILLKKNKHKRAGHGAKNKLKPITILTKKSERFRKKLIERWVCEVADFFIKNKVGTVQMENLESMKRKEDSYFNIRLRGFWPYAEMQNRIEFKLKQYGIEIRKVAPNNTSKTCSKCGHLNSYFNFEYRKKNKFPHFKCEKCNFRENADYNAALNISNPKLRSTKEEP

SEQ ID NO: 2330 - protein, 726 aa, synthetic construct
SEAEFSHEYWMRHALTLAKRARDEREVPVGAVLVLNNRVIGEGWNRAIGLHDPTAHAEIMALRQGGLVMQNYRLTDATLYVTFEPCVMCAGAMIHSRIGRVVFGVRNSKRGAAGSLMNVLNYPDMNHCVEITEGILVDECAALLCDFYRMPRQVLNAQKKAQSSISSGGSSGGSSGSETPGASESATPKSSGGSSASSTKNTITKTLKLRIVRPYNSAKVEKIVADEKNNRERIALEKNKDKVKEACSKHLKVAAYCTTQVERNACLFCRARKLDDKFYQKLRDQFPDAVFWQEIGEIFRQLQRQAAEIYNQSLIELYYEIFIKGKGFANASSVEHYLSDVCYTRAAELFKNAAIASGLRGKVKSNFRLKELKNMKSGLPTTKSDNFPIPLVKQKGGQYTGFEISNHDSDFIIKIPFGRWQAKKEIDKYRPWEKFDFEQVRKSPKPISLLLSTQRRKKNRGWSKDEGTEAEIKKVMNGDYQTSYIEVKRGSKIGEKSAWMLNLSIDVPKIDKGVDPSIIGGIDVGVKSPLVCAISNAFSRYSISDNDLFHFNKKMFARRRILLKKSKHKRAGHGAKNKLKPITILTEKSRRFRKKLIERWACEIADFFIKNKVGTVQMENLESMKRREDSYFNIRLRGFWPYAEMQNKIEFKLKQYGIEIRKVAPNNTSKTCSKCGHLNNYFNFEYRKKNKFPHFKCEKCNFKENADYNAALNISNPKLKGTKEEP

SEQ ID NO: 2331 - protein, 726 aa, synthetic construct
SEVEFSHEYWMRHALTLAKRARDEREVPVGAILVLNNRVIGEGWNRAIGLHDPTAHAEIMALRQGGLVMQNYRLIDATLYVTFEPCVMCAGAMIHSRIGRVVFGVRNSKHGAAGSLMNVLNYPGMNHRVEITEGILADECAALLCDFYRMPRQVFNARKKAQSSINPGGPSGGSSGSGTPDTSESATPESSGGNSGGSAKNTITKTLKLRIVRPYNSAEVEEIVADEKNNREKIALEKNKDKVKEACSKHLKVAAYCTTQVERNACLFCKARRLDDKFYQKLRGQFPDAVFWQEIGEIFRQLQKQAAEVYNQSLVELYYEILIKGKGIANASSVEHYLSDVCYTRAAELFKNAAIASGLRNKIKSNFRLKELRNMKSGLPTTKSDNFPIPLVKQKGGQYTGFEISNHNSDFIIKIPFGRWQVKKEINKYRPWEKFDFEQVRKSPKPISLLLSTQRRKRNKGWSKDEGTEAEIRKVMNGDYQTSYIEVKRGSRIGEKSAWMLSLSIDVPKIDRGVDPSIIGGIDVGVKSPLVCAINNALSRYSISDNDLFHFNKKMFARRRILLKKNRHKRAGHGAKNKLKPLTILTGKSKRFRKKLIERWACEIADFFIKNKVGTVQMENLESMKRKEDSYFNIRLRGFWPYAEMQNRIEFKLKQYGIEIRKVAPNNTSKTCSKCGHLNNHFNFEYRKKNKFPHFKCEKCNFKENADYNAALNISNPKLKSTKGEP

SEQ ID NO: 2332 - protein, 726 aa, synthetic construct
SEDEFSHEYWMRHALTLAKRARDGREVPVGAVLVLNNRVIGEGWNRAIGLHDPTAHAEIMALRQGGLVMQNYRLIDATLYVTFEPCVMCAGAMVHSRIGRVVFGVRNSKRGAAGSLMNVLDYPGMGHRVEITEGILADECAALLCDFYCMPRQVFNAQKRAQSSINPGGSSGGSSVSDTPGTSESATPESSGGGSSGSAKNTVTKTLQLRIVRPYNSAEVEKIVADEKSNREKIALEKNKDKVREACSKHLKVASYCTTQVERNACPFCKARKLDDKFYQKLRGQFPDAVFWQELGEILRQLQKQAAEIYNQSLIELYYEIFIKGKGFANASSVEHYLSDVCYTRAAELFKNAAIASGLRGKVKSNFRLKELKNMKSGLPTTKSDNFPIPLVKQKGGQYAGFEISSHNDDLIIKIPFGRWQVKKEIDKYRPWEKFDFEQVRKSPKPISLLLSTQRRRRNKGWSKDEGTEAEIRKVMNGDYQTSYIEVKRGSKIGEKSAWMLNLSIDVPKIDKGVDPSIIGGIDVGVKSPLVCAINNAFSRYSISDNDLFHFNKKMFARRRILLKKNRHKRAGHGAKNKLKPISILTEKSKRFRKKLIERWACEIADFFIKNKVGTVQMENLESMKRKEDSYFNIRLRGFWPYAEMQNKIEFKLKQYGIEIRKVAPNNTSKTCSRCGHLNNYFNFEYRRKNKFPHFKCEKCNFKENADYNAALNICNPKLKSTKEEP

SEQ ID NO: 2333 - protein, 726 aa, synthetic construct
SEVEFSHEYWMRRALTLAKRARDEREVPVGAVLVLNNRVIGVGWNRAVGLHDPTAHAEIMALRQGGLVMQNYCLVEATLYVTFEPCIMCAGAMIHSRIGRVVFGVRNSKRGAAGSLMNVLNYPGMNHRVEITEGILADECAALLCDYYRMPRQVFNARKKAQSSINPGGSSGGSSGSETPGTSVSATPESSGGSSGGSAKNTITKTLKLRIVRPYNSVEVEKIVADEKNNREKIALEKNKDKVKEACSKHLKVAAYCTTQVERNACLFCKARRLDDKFYQKLRGQFPDAVFWQEIGEIFRQLQKQAAEIYNRSLIELYYEIFIKGKGIANASSVEHYLSDVCYTRAAELFKNAAIASGLRNKVRSNFRLKELKSMKSGLPTTKSDNFPIPLVKQKGGQYTGFEISSHNDDFIIKIPFGRWQVKKEINKFRPWEKFDFEQVRKSPKPISLLLSTQRRKRNKGWSRDEGTEAEIRKVMNGDYQTSYIEVKRGSKTGEKSAWMLNLSIDVPKIDKGVDPSIIGGIDVGVKSPLVCAINNALSRYSISDNDLFHFNKKVFARRRILLRKNRHKRAGHGARNKLKPITVLTEKSERFRKKLIERWACEIANFFIKNKVGTVQMENLESMKRREDSYFNTRLRGFWPYAEMQNKIEFKLKQYGIEIRKVAPNNTSKTCSKCGHLNNYFNFEYRKKNKFPHFKCEKCNFKENADYNAALNISNPKLRSTKEEP

SEQ ID NO: 2334 - protein, 726 aa, synthetic construct
SEVEFSHEYWMRHALALAKRARDEREVPVGAVLVLNNRAIGEGWNRAIGLHDPTAHAEIMALRQGGLVLQNYRLVDATLYVTFEPCVLCAGAMVHSRIGRVVFGARNSKRGAAGSLMNILNYPGMDHRVEITEGILADECAALLCDFYRMPRQVFNAQKKAQSSINSGGSSSGSSGSETPSTSESATPESFGGSSGGSAKNTITKTLKLRIVRPYNSAEVEKIVADEKNNREKIALEKNKDKVKEACSKHLKVASYCTTQVERNACPFCKARKLDDKFYQKLRGQFPDAVFWQELGEIFRQLQKQAAEIYNQSLIELYYEIFIKGKGFANASSVEHYLSDVCYTRAAELFKNAAIASGLRGKVKSNFRLKELKSMKSGLPTTKSDNFPIPLVKQKGGQYTGFEISNRNSDFIIKIPFGRWQVKEEIDKYRPWEKFDFEQVRKSPKPISLLLSTQRRKRNKGWSRDEGTEAEIKKVMNGDYQTSYIEVKRGSKTGEKSAWMLNLSIDVPKIDKGVDPCIIGGIDVGVKSPLVCAINNAFSRYSISDNDLFHFNKKMFARRRILLKKNRHKRAGHGAKNKLKPISILTEKSKRFRKKLIERWACEIADFFIKNKVGTVQMENLESMKRREDSYFNIRLRGFWPYAEMQNKIEFKLKQYGIEVRKVAPNNTSKTCSKCGHLNNYFNFEYRKKNKFPHFKCEKCNFKENADYNAALNISNPKLKSTKEEP

SEQ ID NO: 2335 - protein, 726 aa, synthetic construct
SEVEFSHEYWMRHALTLAKRARDEREVPVGAVLVLNNRVIGEGWNRAIGLHDPTAHAEVMALRQGGLVMQNYRLTDATLYVTFEPCVMCAGAMIHSRIGRVVFGVRNSKRGAAGSLMNVLNYPGMNHCVEITEGILVDECAALLCDFYRMPRQVLNAQKKAQSSISPGDSSGGSSGSETPGASGSVTPKSSGGSSAGSTKNTITKTLKLRIVRPYNSAEVEKIVADEKNSREKIALEKNKDKVKEACSEHLKVAAYCTTQVERSACLFCKARKLDDRFYQKLRGQFPDAVFWQEISEIFRQLQKQAAEIYNQSLIELYYEILIKGKGIANASRVEHYLSDVCYTRAAELFKNAAIASGLRGKVKSNFRLKELKNMKSGLPTTKSDNFPIPLVKQKGGQYTGFEVSSHNDDFIIKIPFGRWQVKKEIDKYRPWEKFDFEQVRKSPRPISLLLSTQRRKRNKGWSKDEGTEAEIRKVMNGDYQTSYIEVKRGSKIGEKSAWMLNLSIDVPKIDKGVDPSIIGGIDVGVKSPLVCAIDNAFSRYSISDNDLFRFNKKVFARRRILLKKNRHKRAGHGTKNKLKPITILTEKSGRFRKKLIERWACEIANFFIKNKVGTVQMENLESMKRKEDSYFNIRLRGFWPYAEMQSKIEFKLKQYGIKIRKVAPNNTSKTCSKCGHLNYYFSFEYRKKNKFPHFKCEKCNFKEDADYNAALNISNPKLKSTKEEP

SEQ ID NO: 2336 - protein, 726 aa, synthetic construct
SEVEFSHEYWMRHALTLAKRARDEREVPVGAVLVLNNRVIGEGWNRAIGLHDPTAHAEIMALRQGGLVMQNHRLVDATLYVTFEPCVLCAGAMVHSRIGHVVFGVRNSKRGAAGSLMNVLNYPGMNHRVEITEGILADECAALLCDFYRMPRQVFNAQKKARSNINSGGSSGSSSGSETPGTSESATPESSGGSSGGSAKNTITKALKLRIVRPYNSAEVERIVADEKNNREKIALEKNKDKVKEACSEHLKVAAYCTTQVERNACLFCKARKLDDEFYQRLRGQFPDAVFWQELGGIFRQLQKQAAEIYNQSLIELYYEIFIKGKGITNASRVEHYLSDVCYTRAAELFKNAAIASGLRSKVRSNFRLKELKNMKSGLPTTKSDNFPIPLVKQKGGQYTGFEISSHNSDFIIKIPFGRWQVKEEIDKYRPWEKFDFEQVRKSPKPISLLLSTQRRKKNKGWSKDEGTEAEIRRVMNGDYQTSYIEVKRGSKIGEKSAWMLNLSIDVPKIDKGVDPSIIGGIDVGVKSPLVCAINNSSSRYSICDNDLFRFNKKMFARRRILLKKNRHKRAGHGAKNKLKPITILTKKSERFRKKLIERWVCEVADFFIKNKVGTVQMENLESMKRKEDSYFNIRLRGFWPYAEMQNKIEFKLKQYGIEIRKVAPNNTSKTCSKCGHLNNYFNFEYRKKNKFPHFKCEKCNFKENADYNAALNISNPRLKSTKEEP

SEQ ID NO: 2337 - protein, 726 aa, synthetic construct
SEDEFSHEYWMRHALTLAKRARDGREVPVGAVLVLNNRVIGEGWNRAIGLHDPTAHAEIMALRQGGLVMQNYRLTDATLYVTFEPCVMCAGAMIHSRIGRVVFGVRNSKRGAAGSLMNVLNYPGMNHRVEITEGILVDECAALLCDFYRMPCQVLNAQKKAQSSISSGGSSGGSSGGDTLGASESVTPKSSVGSSASSTKNTITKTLKLRIVRPYNSAEVEKIVADEKNNREKIALEKNKDKVKEACSKHLKVAAYCTTQVERNACLFCKARRLDDKFYQKLRGQFPDAVFWQELGEIFRQLQKQAAEIYNQSLIELYYEIFIKGKGFANASSVEHYLSDVCYTRAAELFKNAAIASGLRGKVKSNFKLKELKSMKSGLPSTKSDNFPIPLVKQKGGQYTGFEISSHNDDFIIKIPFGRWQVKKEIDKYRPWEKFDFEQVRKSPKPISLLLSTQRRKRNKGWSKDEGTEAEIRKVMNGDYRTSYIEVKRGSKTGEKSAWMLNLSIDVPKIDKGVDPSIIGGIDVGVKSPLVCAINNAFSRYSISDNDLFRFNKKMFARRRILLRKNRHKRAGHGAKNKLKPITILTEKSVRFRRKLIERWACEIADFFVKNKVGTVQMENLESMKRKEDSYFNIRLRGFWPYAEMQNKIEFKLKQYGIEIRKVAPNNTSRTCSKCGHLNDYFNFEYRKKNKFPHFKCEKCSFKENADYNAALNISNPKLKSTKEEL

SEQ ID NO: 2338 - protein, 726 aa, synthetic construct
SEVEFSHEYWMRHALTLAKRARDEREVPVGAVLVLNNRVIGEGWNRTTGLHDPTAHAEIMALRQGGLVMRNYRLTDATLYVTFEPCVMCAGAMIHSRIGRVVFGVRNSKRGAAGSLMNVLNYPGMNHCVEITEGILVDECAALLCDFYRMPRQVLNAQRRAQSSISPGGSSGGSSGSEAPGASESVTPKNSGGSSGGSAKNTITKTLKLRIVRPYNSAEVEKIVADEKNNREKIALEKNKGKVKEACSKHLEVAAYCTTQVERNACLFCKARKLDDKFYQKLRGQFPDAVFWQELGEIFRQLQKQAAEIYNQSLIELYYEIFIKGKGITNASRVEHYLSDVCYTRAAELFKNAAIASGLRSKVRSNFRLKELKSMKSGLPTTKSDNFPIPLVKQKGGQYTGFEISSHNSDFIIKIPFGRWQVKKEIDKYRPWEKFDFEQVRKSPKPISLLLSTQRRKRNKGWSKDEGTEAEIRKVMNGDYQTSYIEVKRGSRIGEKSAWMLNLSIDVPKIDKGVDPSNIGGIDVGVKSPLVCAINNAFSRYSISDNDLFHFNKKMFARRRILLKKNGHKRAGHGAKNKLKPISILTEKSERFRKKLIERWACEIADFFIKNKVGTVQMENLESMKRREDSYFNTRLRGFWPYAEMQNKIEFKLKQYGIEIRKVAPNNTSRTCSKCGHLNNYFNFEYRKKNKFPHFKCEKCNFKENADYNAALNICNPKLKSTKEEP

SEQ ID NO: 2339 - protein, 726 aa, synthetic construct
SEDEFSHEYWMRHALTLAKRARDEREVPVGAILVLNNRVIGEGWNRAIGLHDPTAHAEIMALRQGGLVMQNYRLIDATLYVTFEPCVMCAGAMIHSRIGRVVFGVRNNKHGAAGSLVNVLNYPGMNHRVEITEGILADECAALLCDFYRMPRQVFNARKKAQSSINPGGSSGGSSGSETPGTSESATPESSGGSSGGSAKNTITKTLKLRIVRPYNSAEVEKIVADEKNNREKIALEKNKDKVKEACSKHLKVAAYCTTQVERNACLFCKARKLDDKFYQKLRGQFPDAVFWQEIGEIFRQLQKQAAEIYNQSLIELYYEIFIKGKGFANASSVEHYLSDVCYTRAAELFKNAAIASGLRGKVKSNFRLKELKNMKSGLPTTKSDNFPIPLVKQKGGQYTGFEISSHNDDFIIKIPFGRWQVKKEIDKYRPWEKFDFEQVRKSPKPISLLLSTQRRKRNKGWSKDEGTEAEIRKVMNGDYQTSYIEVKRGSKTGEKSAWMLNLSIDVPKIDKGVDPSIIGGIDVGVKSPLVCAINNAFSRYSISDNDLFRFNKKMFARRRILLKKNRHKRAGHGAKNKLKPISILTGKSERFRKKLIERWACEIADFFIKNKVGTVQMENLDSMKRKEDSYFNIRLRGFWPYAEMQNKIESKLKQYGIEIRKVAPNNTSKTCSKCGHLNNYFNFEYRKKNKFPHFKCEKCNFKENADYNAALNISNPKLKSTKEEP

SEQ ID NO: 2340 - protein, 726 aa, synthetic construct; identical to SEQ ID NO: 684

SEQ ID NO: 2341 - protein, 726 aa, synthetic construct
SEVEFSHEYWMRHALTLAKRARDEREVPVGAVLVLNNRVIGEGWNRAIGLHDPTAHAEIMALRQGGLVMQDYRLTDATLYVTFEPCVMCAGAMIHSRIGRVVFGVRNSKRGAAGSLMNVLNYPGMNHCVEITEGILVDECAALLCDFYRMPRQVLNAQKKAQSSISSGGSSGGSSGSETPGASGSVTPGSSGGSSGGSAKNTITKTLKLRIVRPYNSAEVEKIVADEKNSREKIALEKNKDKVKEACSEHLKVAAYCTTQVERNACLFCKARKLDDRFYQKLRGQFPDAVFWQETGEIFRQLQKQAAEIYNQSLIELYYEILIKGKGFANASSVEHYLSDVCYTRAAELFKNAAIASGLRGKVKSNFRLKELKNMKSGLPTTKSDNFPIPLVKQKGGQYTGFEISSHHDDFIIKIPFGRWQVKKEIDKYRPWEKFDFEQVRKSPKPISLLLSTQRRKRNKGWSKDEGTEAEIRKVMNGDYQTSYIEVKRGSKIGEKSAWMLSLSIDVPKIDKGVDPSIIGGIDVGVKSPLVCAINNALSRYSISDNDLFHFNKKMFARRRILLKKNRHKRAGHGARNKLKPFTILTEKSVRFRKKLIERWACEIANFFIKNKVGTVQMENLESMKRKEDSYFNIRLRGFWPYAEMQNKIEFKLKQYGITIRRVAPNNTSKTCSKCGHLNNYFSFEYRKRNKFPHFKCEKCNFKEDADYNAALNISNPKLKSTKEEP

SEQ ID NO: 2342 - protein, 726 aa, synthetic construct; identical to SEQ ID NO: 684

SEQ ID NO: 2343 - protein, 726 aa, synthetic construct
SEVEFSHEYWMRHALTLAKRARDEREVPVGAVLVLNNRVIGVGWNRAIGLHDPTAHAEIMALRQGGLVMQNYRLIGATLYVTFEPCAMCAGAMIHSRIGRVVFGVRNSKRGAAGSLMNVLNYPGMNHRVEIMEGILTDECAALLCDFYHMPHQVLNAQKKAQSSINSGGSSGGSSGSETPGASGSVTPKSSVGSSAGSTKNTITKTLKLRIVRPYNSAEVEKIVADEKNNREKIALEKNKDKVKEACSEHLKVAAYCTTQVERNACLFCKARKLDDKFYQKLRGQFPDAVFWQEIGEIFRQLQKQAAEIYNQSLIELYYEIFIKGKGFANASSVEHYLSDVCYTRAAELFKNAAIASGLRGKVKSNFRLKELKNMKSGLPTTKGDNFPIPLVKQKGGQYTGFEISSHNDDFIIKIPFGRWQVKKEIDKYRPWEKFDFEQVRKSPKPISLLLSTQRRKRNKGWSKDEGTEAEIRKVMNGDYQTSYIEVKRGRKIGEKSAWMLNLSIDVPKIDKGVDPSTIGGIDVGVKSPLVCAINNAFSRHSISDNDLFRFNKKMFARRRILLKKNRHKRAGHGAKNKLKPVTILTEKSGRFRKKLIERWACEIADFFIKNKVGTVQMENLESMRRREDSYFNIRLRGFWPYAEMQNKIEFKLKQYGIRIRKVAPNNTSKTCSVCGHLNNYFNFEYRKKNKFPHFKCEKCNFKENADYNAALNISNPKLKSTKEEP

SEQ ID NO: 2344 - protein, 726 aa, synthetic construct
SEDEFSHEYWMRHALTLAKRARDGREVPVGAVLVLNNRVIGEGWNRAIGLHDPTAHAEIMALRQGGLVMQNYRLIDATLYVTFEPCVMCAGAMVHSRIGRVVFGVRNSKRGAAGSLMNVLSYPGMNHRVEITEGILADECAALLCDFYRMPRRVFNAQKKAQSSINSGGSSGGGSGSETPGTSESPTPESPGGSSGGSAKNTITKTLKLRIVRPYNSAEVEKIVADEKNNREKIALEKNKDKVKEACSKHLKVAAYCTTQVERNACLFCKARKLDDKFYQKLRGQFPDAVFWQEIGEIFRQLQKQAAEIYNQSLIELYYEIFIKGKGFANASSVEHYLSDVCYTRAAELFKNAAIASGLRGKVKSNFRLKELKNMKSGLPTTKSDNFPIPLVKQKGGQYTGFEISSHNDDFIIKIPFGRWQVKKEIDKYRPWEKFDFEQVRKSPKPISLLLSTQRRKRNKGWGKDEGTEAEIRKVMNGDYQTSYIEVKRGSKIGEKSAWMLNLSIDVPKIDKGVDPSIIGGIDVGVKSPLVCAINNALSRYSISDNDLFHFNKKMFARRRILLRKNRHKRAGHGARNKLKPITVLTEKSERFRKKLIERWACEIANFFIKNKVGTVQMENLESMKRREDSYFNIRLRGFWPYAEMQNKIEFKLKQYGIEIRKVAPNNTSKTCSKCGHLNNYFNFEFRKKNKFPHFKCEKCNFKENADYNAALNISNPKLKSTKEEP

SEQ ID NO: 2345 - protein, 726 aa, synthetic construct; identical to SEQ ID NO: 684

SEQ ID NO: 2346 - protein, 726 aa, synthetic construct
SEVEFSHEYWMRHALTLAKRARDEREVPVGAVLVLNNRVIGEGWNRTTGLHDPTAHAEIMALRQGGLVMRNYRLTDATLYVTFEPCVMCAGAMIHSRIGRVVFGVRNSKRGAAGSLMNVLNYPGMNHCVEVTEGILVDECAALLCDFYRMPRQVLNAQKKAQSSISPGGSSGGSSGSETPGASGSVTPKSSGGSSAGSTKDTITKTLKLRIVRPYNSAEVEKIVADEKNSREKIALEKNKDKVKEACSEHLKVAAYCTTQVERSACLFCKARKLDDKFYQRLGGQFPDAVFWQEIGEIFRQLQKQAAEIYNQSLIELYYEIFIKGKGFANASSVEHYLSDVCYTRAAELFKNAAIASGLRSKIKSNFRLKELRNMKSGLPTTMSDNFPIPLVKQKGGQYTGFEISNHNGDFIIKIPFGRWQVKKEIDKYRPWEKFDFEQVRKSPKPISLLLSTQRRKRSKGWSKDEGTEAEIRKVMNGDYQTSYIEVKRGSKIGEKSAWMLNLSIDVPKIDKGVDPSIIGGIDVGVKSPLVCAINNAFSRYSISDNDLFRFNKKMFARRRILLGKNRHKRAGHGVKNKLKPITILTEKSGRFRKKLIERWACEIADFFVKNKVGTVQMENLESMKRKEDSYFNIRLRGFWPYAEMQNKIEFKLKQYGIKIRKVAPHNTSKTCSKCGHLNNYFSFEYRKKNKFPHFRCEKCNFKENADYNAALNISNPKLKSTKEEP

SEQ ID NO: 2347 - protein, 726 aa, synthetic construct
SEAEFSHEYWMRRALTLAKRARDEREVPVGAVLVLNNRVIGVGWNRAVGLHDPTAHAEIMALRQGGLVMQNYRLVEATLYVTFEPCIMCAGAMIHSRIGRVVFGVRNSKRGAAGSLMNVLNHPGMNHRVEITEGILADECAALLCDYYRMPRQVFNARKKAQPSINSGGSSGGNSGSETPGSSESATPESSGGSSGGTAKDTITKTLKLRIVRPYNSAEVEKIVADEKNNRERIALEKNRDKVKEACSKHLKVAAYCTTQVERNACLFCKARKLDDKFYQKLRGQFPDAVFWQEIGEIFRQLQKQAAEIYNQSLIELYYEIFIKGKGFANASSVEHYLSDVCYARAAELFKNAAIASGLRGKVKSNFRLKELKNMKSGLPTTKSDNFPIPLVKQKGGQYTGFEISNHNDDFIIKIPFGRWQVKEEIDKYRPWEKFDFEQVRKNPKPISLLLSTQRRKGNKGWSKDEGTEAEIRKVMNGDYQTSYIEVKRGSKIGEKSAWMLNLSIDVPKIDKGVDPSIIGGIDVGVKSPLVCAINNAFSRYSISDNDLFHFNKKMFARRRILLKKNRHRRAGHGAKNKLKPISILTEKSKRFRKKLIERWACEIADFFIKNKVGTVQMENLESMKRKEDSYFNIRLRGLWPYAEMQNKIEFKLKQYGIEIRKVAPNNTSKTCSKCGHLNNYFNFEYRKRNKFPHFKCEKCNFKENADYNAALNISNPKLKGTKEEP

SEQ ID NO: 2348 - protein, 726 aa, synthetic construct
SEVEFSHEYWMRHALTLAKRARDEREVPVGAVLVLNNRVIGEGWNRAIGLHDPTAHAEIMALRQGGLVMQNYRLVNATLYVTFEPCVMCAGAMIHSRIGRVAFGVRNSKRGAAGSLMNVLSYPGMNHRVEITEGILAGECAALLCDFYRMPRQVFNARKKAQSNISSGGSSGGSSGSETPGTCGSPTPESSSGSSGGSAKNTITKTLKLRIVRPYNSAVVEKIVADEKNNREKIALEKNKDKVKEACSKHLKVAAYCTTQVERNACLFCKARKLDDKFYQKLRGQFPDAVFWQEIGEIFRQLQKQAAEIYNQSLIELYYEIFIKGKGFANASSVEHYLSDVCYTRAAELFKNAAIASGLRGKVKSNFRLKELKNMRSGLPTTKSDNFPIPLVRQKGGQYTGFEISSHNDDFVIKIPFGRWQVKKEIDKYRPWEKFDFEQVRKSPKPISLLLSTQRRKRNKGWSKDEGTEAEIRKVMNGDYQTSYIEVKRGSKNGEKSAWTLNLSIDVPKIDKGVDPSIIGGIDVGVKSPLVCAINNAFSRYSISDNDLFRFNKKMFARRRILLKKNRHKRAGHGVKNKLKPISILTGKSERFRRKLIERWACEIADFFIKNKVGTVQMENLGSMKRREDSYFNIRLRGFWPYAEMQNKIEFKLKQYGIEIRKVAPNNTSKTCSRCGHLNNYFNFEYRKRNKFPHFKCEKCNFKENADYNAALNISNPKLKSPKEEP

SEQ ID NO: 2349 - protein, 726 aa, synthetic construct
SEDEFSHEYWMRHALTLAKRARDGREVPVGAVLVLNNRVIGEGWNRAIGLHDPTAHAEIMALRQGGLVMQNYRLIDATLYVTFEPCVMCAGAMVHSRIGRVVFGVRNSKRGAAGSLMNVLDYPGMDHRVEITEGILADECAALLCDFYRMPRQVFNAQKKAQSSINSGGSSGGSSGSETPGTSESATPESSGGGSSGSAKNTITKTLQLRIVRPYNSAEVEKIVADEKNNREKIALEKNKDKVKEACSKHLKVASYCTTQVERNACPFCKARKLDDKFYQKLRGQFPDAVFWQELGEILRQLQKQAAEIYNQSLIELYYEIFIKGRGFANASSVEHYLSDVCYTRAAELFKNAAIASGLRGKVKGNFRLKELKNMKSGLPTTKSDNFPIPLVKQKGGQYTGFEISSHNDDFIIKIPFGRWQVKKEIDKYRPWEKFDFEQVRKSPKPISLLLSTQRRKRNKGWSRDEGTEAEIRKVMNGDYQTSYIEVKRGSKTGEKSAWMLNLSIDVPKIDKGVDPCIIGGIDVGVKSPLVCAINNAFSRYSISDNDLFHFNKKMFARRRILLKENGHKRAGHGAKNKLKPITIMTEKSKRFRKKLIERWACEIADFFIKNKVGTVQMENLESMKRKEDSYFNIRLRGFWPYAEMQNKIEFKLKQYGIKIRKVAPNNTSKTCSKCGHLNNYFSFEYRKKNKFPHFKCEKCNFKENADYNAALNISNPKLKSTKEEP

SEQ ID NO: 2350 - protein, 726 aa, synthetic construct
SEVEFSHEYWMRHALTLAKRARDEREVPVGAVLVLNNRVIGEGWNRAIGLHDPTAHAEIMALRQGGLVMQNYRLTDATLYVTFEPCVMCAGAMIHSRIGRVVFGIRNSKRGAAGSLMNVLNYPGMNHCVEITEGILVDECAALLCDFYRMPRQVLNAQKKAQSSISSGGSSGGSSCSETPGASESVTPKSSGGSSGGSAKNTITKTLKLRIVRPYNSAEVEKIVADEKDNREKIALEKNKDKVKEACREHLKVAAYCTTQVERSACLFCKARKLDDKFYQKLRGQFPDAVFWQELGEILRQLQKQAAEIYNQSLIELYYEIFIRGKGIASTSRVGHYLSDVCYTRAAELFKNAAIASGLRSKIKSNFRLKELKNMKSGLPTTKSDNFPIPLVKQKGGQYTGFEISSHNDDFIIKIPFGRWQEKKEINKYRPWEKFDFEQVRKSPKPISLLLSTQRRKRNKGWSKDEGTEAEIRKVLNGDYQTSYIEVKRGSKTGEKSAWMLNLSIDVPKIDKGVDPSIIGGIDVGVKSPLVCAINNALSRYSISDNDLFHFNKKMFARRRILLRKNRHKRAGHGARNKLKPITVLTEKSERFRKKLIERWACEIANFFIKNKVGTVQMENLESMKRREDSYFNIRLRGFWPYAEMQSKIEFKLKQCGIKIRKVAPNNTSKTCSKCGHLNNYFNFEFRKKNKFPHFKCEKCNFKENADYNAALNISNPMLKSTKEEP

SEQ ID NO: 2351 - protein, 726 aa, synthetic construct; identical to SEQ ID NO: 684

SEQ ID NO: 2352 - protein, 726 aa, synthetic construct
SEVEFNHEYWMRHALTLAKRARDGREVPVGAVLVLNNRVIGEGWNRAIGLHDPTAHAEIMALRQGGLVMQNYRLIDATLYVTFEPCVMCAGAMVHSRIGRVVFGVRNSKRGAAGSLMNVLDYPGMGHRVEITEGILAGECAALLCDFYRMPRQVFNAQKKAQSNINSGGSSGGSSGSETLGTSESATPESSGGSSGGSAKNTITKTLKLRIVRPYNSAEVEKIVADEKNNREKIALEKNKDKVKEACSEHLKVAAYCTTQVERNACPFCKARKLDDKFYQKLRGQFPDAVFWQEISEIFRQLQKQAAEIYNQSLVELYYEIFIKGKGIANASSVEHYLSDVCYTRAAELFKNAAIASGLRNKIKSNFRLKELRNMKSGLPTTKSDNFPIPLVRQKGGQYTGFEISNHNGDFIIKIPFGRWQVKKEISKHRPWEKFDFEQVRKSPKPISLLLSTQRRKRNKGWGKDEGTEAEIRKVMNGDYQTSYIEVKRGSKVGEKSAWMLNLSIDVPKIDKGVDPSIIGGIDVGVKSPLVCAINNALSRYSISDNDLFHFNKKMFARRRILLRKNRHKRAGHGARNKLKPITVLTEKSERFRKKLIERWACEIADFFIKNKVGTVQMENLEGMKRKEDSYFNIRLRGFWPYAEMQNKIEFKLKQYGIEIRKVVPNNTSKTCSKCGHLNNYFSFEYRKKYKFPHFKCEKCNFKEDADYNAALNISNPMLKSTKEEP

SEQ ID NO: 2353 - protein, 726 aa, synthetic construct
SEVEFSHEYWMRHALTLAKRARDEREVPVGAVLVLNNRVIGEGWNRAIGLHDPTAHAEIMALRQGGLVMQNHRLVDATLYVTFEPCVMCAGAMIHSRIGRVVFGVRNSKRGAAGSLTNVLNYPGMNHRVEITEGILVDECAALLCDFYRMPRQVFNARKKAQSTINSGGSSGGSSGSETPGTSESPTPESSGGSPGGSAKNTITKTLKLRIVRPYNSAEVEKIVADEKNNREKIALEKNKDKVKEACSKHLKVAAYCTTQVGRNACLFCKARRLDDKFYQKLRGQFPDAVFWQEIGEIFRQLQKQAAEVYNQSLVELYYEIFIKGKGLANASSVEHYLSDVCYTRAAELFKNAAIASGLRGKVKSNFKLKELKSMKSGLPSTKSDNFPIPLVKQRGGQYTGFEISSHNDDFIIKIPFGRWQAKKEIDKYRPWEKFDFEQVRKSPKPISLLLSTQRRKRNRGWSKDEGTEAEIRKVMNGDYQTSYIEVKRGSKIGEKSAWMLNLSIDVPKIDKGVDPSIIGGIDVGVKSPLVCAINNAFSRYSISDNDLFRFNKKMFARRRILLGKNRHKRAGHGVKNKLKPITILTEKSGRFRKKLIERWACEIADFFVKNKVGTVQMENLESMKRKEDSYFNIRLRGFWPYAEMQNKIEFKLKQYGIKVRKVAPNNTSKTCSKCGHLNNYFSFEYRKKNKFPHFKCEKCNFKENADYNAALNISNPKLKSTKEEP

SEQ ID NO: 2354 - protein, 726 aa, synthetic construct
SEGEFSHEYWMRHALTLAKRARDGREVPVGAVLVLNNRVIGEGWNRAIGLHDPTAHAEIMALRQGGLVMQNYRLFDATLYVTFEPCVMCAGAMVHSRIGRVVFGVRNSKHGAAGSLMNVLNYPGMNHRVEITEGILADECAALLCDFYRMPHQVFNARKKAQSSIDPSGSSGGSSGSVTPGTSESATPESSGGGFGGSAKNTITKTLQLRIVRPYNSAEVEKIVADEKNNREKIALEKNKDKVKEACSKHLKVASYCTTQVERNACLFCKARKLDDKFYQKLRGQFPDAVFWQELGEIFRQLQKQAAEIYNQSLIELYYEIFIKGKGITNASRVEHYLSDVCYTRAAELFKNAAIASGLRSKVRSNFRLKELKNMKSGLPTTKSDNFPIPLVKQKGGQYTGFEISSHNSDFIIKIPFGRWQMKEEIDKYRPWEKFDFEQVRKSPKPISLLLSTQRRKKNKGWSKDEGTEAEIRRVMNGDYQTSYIEVKRGSKIGEKSAWMLNLSIDVPKIDKGVDPSIIGGIDVGVKSPLVCAINNSSSRYSICDNDLFRFNKKMFARRRILLKKNRHKRAGHGAKNKLKPITILTKKSERFRKKLIERWVCEVADFFIKNKVGTVQMENLESMKRKEDSYFNIRLRGFWPYAEMQNKIEFKLKQYGIVVRKVAPNNTSKTCSQCGHLNNYFNFEYRKKNKFPHFKCEKCNFKENADYNAALNISNPRLKSTKEEP

SEQ ID NO: 2355 - protein, 726 aa, synthetic construct
SEDEFSHEYWMRHALTLAKRARDGREVPVGAVLVLNNRVIGEGWNRAIGLHDPTAHAEIMALRQGGLVMQNYRLIDATLYVTFEPCVMCAGAMVHSRIGRVVFGVRNSKRGAAGSLMNVLDYPGMGHRVEITEGILADECAALLCDFYCMPRQVFNAQKRAQSSINSGGSSGGSCGSDTPGTSESATPESSGGGSSGSAKNTITKTLQLRIVRPYNSAEVEKIVADEKNNREKIALEKNKDKVREACSKHLKVASYCTTQVERNACPFCKARKLDDKFYQKLRGQFPDAVFWQELGEILRQLQKQAAEIYNQSLIELYYEIFIKGRGFANASSVEHYLSDVCYTRAAELFKNAAIASGLRGKVKGNFRLKELKNMKSGLPTTKSDNFPIPLVRQKGGQYTGFEISSHNDDFIIKIPFGRWQVKKEIDKYRPWEKFDFEQVRKSPKPISLLLSTQRRKRNKGWSKDEGTEAEIRKVMNGDYQTSYIEVKRGSRTGEKSAWMLNLSIDVPKIDKGVDPSIIGGIDVGVKSPLVCAINNAFSRYSISDNDLFRFNKKMFARRRILLKKNRHKRAGHGAKNKLKPISILTGKSERFRKKLIERWACEIADFFTKNKVGTVQMENLESMKRKEDSYFNIRLRGFWPYAEMQNKIEFKLKQYGIEIRKVAPNNTSKTCSKCGHLNNYFNFEYRKKNKFPHFRCEKCNFKENADYNAALNISNPKLKSTKEEP

SEQ ID NO: 2356 - protein, 726 aa, synthetic construct
SEVEFSHEYWMRHALTLAKRARDEREVPVGAILVLNNRVIGEGWNRAIGLHDPTAHAEIMAMRQGGLVLQNYRLIDATLYVTFEPCVMCAGAMIHSRIGRVVFGVRNNKHGAAGSLVNVLNYPGMNHRVEITEGILADECAALLCDFYRMPRQVFNARKKAQSSINPGGSSGGSSGSETPGTSESATPGSSGGSSGSSAKNTITKTLKLRIVRPYNSAEVEKIVADEKNNREKIALEKNKDKVKEACGKHLKVAAYCTTQVERNACLFCKARRLDDKFYQKLRGQFPDAVFWQEIGEIFRQLQKQAAEIYNQSLIELYYEIFIKGKGFANASSVEHYLSDVCYTRAAELFKNAAIASGLRGKVKSNFRLKELKNMKSGLPTTKSDNFPVPLVKQKGGQYTGFEISNHNSDFIIKIPFGRWQVKEEINKYRPWEKFDFEQVRKSPKPISLLLSTQRRKRNKGWSKDEGTEAEIRKVMNGDYQTSYIEVKRGSKTGEKSAWMLNLSIDVPKIDKGVDPSIIGGIDVGVKSPLVCAINNAFSRYSISDNDLFRFNKKMFARRRILLKKNRHKRAGHGAKNKLKPISILTGKSERFRKKLIERWACEIADFFIKNKVGTVQMENLESMKRRGDSYFNIRLRGFWPYAEMQNKIEFKLKQYGIEIRKVAPNNTSKTCSKCGHLNNYFNFEYRRKNKFPHFKCEKCNFKEDADYNAALNISNPKLKSTKEEP

SEQ ID NO: 2357 - protein, 726 aa, synthetic construct; identical to SEQ ID NO: 684

SEQ ID NO: 2358 - protein, 726 aa, synthetic construct
SEVEFSHEYWMRHALTLAKRARDEREVPVGAILVLNNRVIGEGWNRAIGLHDPTAHAEIMALRQGGLVMQNYRLTDATLYVTFEPCVMCAGAMIHSRIGRVVFGVRNSKRGAAGSLMNVLNYPGMNHCVEITEGILVDECAALLCDFYRMPRQVLNAQKKAQSSINSGGSSGGSSGSETPGTSESATPESSGGGSSGSAKSTITKTLQLRIVRPYNSAEVEKIVADEKNNREKIALEKNKDKVKEACSKHLKVASYCTTQVERNACPFCKARKLDDKFYQKLRGQFPDAVFWQELGEILRQLQKQAAEIYNQSLIELYYEIFIKGKGFANASSVEHYLSDVCYTRAAELFKNAAIASGLRGKVKSNFRLKELKNMKSGLPTTKSDNFPIPLVKQKGGQYTGFEISSHNDDFIIKIPFGRWQVRKEIDKYRPWEKFNFEQVRKSPKPISLLLSTQRRKRNKGWSKDEGTEAEIRKVMNGDYQTSYIEVKRGSKIGEKSAWMLSLSIDVPKIDKGVDPSIIGGIDVGVKSPLVCAINNAFNRYSISDNNLFHFNKKMFARRRILLKKNRHKRAGHGAKNKLKPISILTEKSERFRKKLIERWACEIADFFIKNKVGTVQMENLESMKRKEDSYFNIRLRGFWPYAEMQNKIEFKLKQYGIEIRKVAPNNTSKTCSKCGHLNNYFNFEYRKKNKFPHFKCEKCNFKENADYNAALNISNPKLKSTKEEP

SEQ ID NO: 2359 - protein, 725 aa, synthetic construct
SEVEFSHEYWMRHALTLAKRARDEREVPVGAVLVLNNRVIGEGWNRAIGLHDPTAHAEIMALRQGGLVMQNYRLSDATLYVTFEPCVMCAGAMIHSRIGRVVFGVRNSKRGAAGSLMNVLNYPGMNHCVEITEGILVDECAALLCDFYRMPRQVLSAQKKAQSSVSSGGSSGGSSGSETPGASGSVTPKSSGGGSSGSAKNTITKTLQLRIVRPYNSAEVEKIVADEKNNREKIALEKNKDKVREACNKHLKVASYCTTQVERNACLFCKARKLDDKFYQKLRGQFPDAVFWQELGEILRQLQKQAAGIYNQSLIELYYEIFIKGKGIANASSVEHYLSDVCYTRAAELFKNAAIASGLRNKIKSNFRLKELRNMKSGLPTTKSDNFPIPLVRQKGGRYTGFEISNHNGDFIIKIPFGRWQVKKEVNKHRPWEKFDFEQVRKSPKPISLLLSTQRRKRNKGWSKDEGTEAEIRKVMNGDYQTSYIEVKRGSKIGEKSAWMLNLSIDVPKIDKGVDPSIIGGIDVGVKSPLVCAINNAFSRYSISDNDLFRFNKKMFARRRILLGKNRHKRAGHGVKNKLKPITILTEKSGRFRKKLIERWACEIADFFVKNKVGTVQMENLESMKRKEDSYFNIRLRGFWPYAEMNKIEFKLKQYGIKVRKVAPNNTSKTCSKCGHLNNYFSFEYRKKNKFPHFKCEKCNFKENADYNAALNISNPKLKSTKEEL

SEQ ID NO: 2360 - protein, 726 aa, synthetic construct
SEVEFSHEYWMRHALTLAKRARDEREVPVGAILVLNNRVIGEGWNRAIGLHDPTAHAEIMALRQGGLVMQNYRLIDATLYVTFEPCVMCAGAMIHSRIGRVVFGVRNSKHGAAGSLMNVLNYPGMNHRVEITEGILVDECAALLCDFYRMPRQVFNARKKAQSSINPGGSSGGSSGSEMPGTSESATPGSSGGGSSGSAKNTITKTLQLRIVRPYNSAEVEKIVADEKNNREKIALEKNKDKVKEACSKHLKVAAYCTTQVERNACLFCKARKLDDKFYQKLRGQFPDAVFWQEIGEIFRQLQKQAAEIYNQSLIELYYEIFIKGKGFANASSVEHYLSDVCYSRAAELFKNAAVASGLRGKVKSNFRLKELKNMKSGLPTTKSDNFPIPLVKQKGGQYTGFEISSHNDDFIIKIPFGRWQVKKEIDKYRPWEKFDFEQVRKSPKPISLLLSTQRRKRNKGWSKDEGTEAEIRKVMNGDYQTSYIEVKRGSKAGEKSAWMLNLSIDVPKIDKGVDPSIIGGIDVGVKSPLVCAINNAFNRYSISDNNLFHFNKKMFARRRILLKKNRHKRAGHGAKNKLKPISILTEKSERFRKKLIERWACEIADFFIRNKVGTVQMENLEGMKRKEDSYFNIRLRGLWPYAEMQNKIEFKLKQYGIEVRKVAPNNTSKTCSKCGHLNNYFNFEYRKKNKFPHFKCEKCSFKENADYNAALNISNPKLKSAKEEP

SEQ ID NO: 2361 - protein, 726 aa, synthetic construct
SEVEFSHEYWMRHALTLAKRARDEREVPVGAILVLNNRVIGEGWNRAIGLHDPTAHAEIMALRQGGLVMQNYRLIDATLYVTFEPCVMCAGAMIHSRIGRVVFGVRNNKHGAAGSLVNVLNYPGMNHRVGITEGILADECAALLCDFYRMTRQVFNARKKAQSSINPGGSSGGSSGSETPGASESVTPKSSGGSSAGSTKNTITKTLKLRIVRPYNSAEVEKIVADEKNSREKFALERNKDKVKEACSEHLKVAAYCTTQVERNACLFCKARKLDDRFYQKLRGQFPDAVFWQETGEIFRQLQRQAAEIYNQSLIELYYEIFIKGKGFANASSVEHYLSDVCYTRAAELFKNAAIASGLRGKVKSNFRLKELKNMRSGLPTTKSDNFPIPLVKQKGGQYAGFEISSHNDDFIIKIPFGRWQVKKEIDKYRPWEKFDFEQVRKSPKPISLLLSTRRRKRNKGWSKDEGTEAEIRKVMNGDYQTSYIEVKRGSKIGEKSAWMLNLSIDVPKIDKGVDPSIIGGIDVGVKSPLVCAINNAFGRYSISDNDLFHFNKKMFARRRILLKKSKHKRAGHGAKNKLKPITIMTEKSKRFRKKLIERWACEIADFFIKNKVGTVQMENLESMKRKEDSYFNIRLRGFWPYAEMQNKIEFKLKQYGIVVRKVAPNNTSKTCSQCGHLNNYFNFEYRKKNKFPYFKCEKCNFKENADYNAALNISNPQLKSTKGEP

SEQ ID NO: 2362 - protein, 726 aa, synthetic construct
SEVEFSHEYWMRHALTLAKRARDEREVPVGAVLVLNNRVIGEGWNRAIGLHDPTAHAEIMALRQGGLVMQNYRLSDATLYVTFEPCVMCAGAMIHSRIGRVVFGVRNSKRGAAGSLMNVLNYPGMNHCVEITEGILVDECAALLCDFYRMPRQVLSAQKKAQSSISSGGSSGGSSGSETPGTSGSVTPKSSVGSSAGSTKNTITKTLKLRIVRPYNSAEVEKIVADEKNNREKIALEKNKGKVKEACSKHLEVAAYCTTQVERNACLFCKARKLDDKFYQKLRGQFPDAVFWQELGEIFRQLQKQAAEIYNQSLIELYYEIFIKGKGFANASSVEHYLSDVCYTRAAELFKNAAIASGLRGKVKSNFRLKELKNMKSGLPTTKSDNFPIPLVKQKGGQYTGFEISSHSDDFIIKIPFGRWQVKKEIDKYRPWEKFDFEQVRKNPKPISLLLSTQRRKRNKGWSKDEGTEAEIRRVMNGDYQTSYIEVKRGSKIGEKSTWMLNLSIDVPKIDKGVDPSIIGGIDVGVKSPLVCAINNAFSRYSISDNDLFRFNKKVFARRRILLKKNRHKRAGHGTKNKLKPITILTEKSGRFRKKLIERWACEIANFFIKNKVGTVQMENLESMKRKEDSYFNIRLRGFWPYAEMQNKIEFKLKQYGIEIRKVAPNNTSKTCSKCGHLNNYFNFEYRKMNKFPHFKCEMCNFKENADYNAALNISNPKLKSTKEEP

SEQ ID NO: 2363 - protein, 726 aa, synthetic construct
SEVEFSHEYWMRHALTLAKRARDEREVPVGAVLVLNNRVIGEGWNRAIGLHDPTAHAEIMALRQGGLVMQNYRLVDATLYVTFEPCVLCAGAMVHSRIGRVVFGVRNNKRGAAGSLMNVLNYPGMNHRVEITEGILADECAALLCDFYRMPRQVFNARKKAQSSINPSGSSGGSSGSVTPGTSESATPESSGGGSSGSAKNTITKTLQLRIVRPYNSAEVEKIVADEKNNRERIALEKNKDKVKEACSKHLKVAAYCTTQVERNACLFCKARKLDDKFYQKLRGQFPDAVFWQETGEIFRQLQRQAAEIYNQSLIELYYEIFIKGKGFANASSVEHYLSDVCYTRAAELFKNAAIASGLRGKVKGNFRLKELKNMKSGLPTTMSGNFPIPLVKQKGGQYTGFEISSHNDDFIIKIPFGRWQAKKEIDKYRPWEKFDFEQVRKSPKPISLLLSTQRRKRNKGWSKDEGTEAEIRKVMNGDYQTSYIEVKRGSKIGEKSAWMLNLSIDVPKIDKGVDPSIIGGIDVGVKSPLVCAINNAFSRYSISDNDLFHFNKKMFARRRILLKKNRHKRAGHGAKNKLKPISILTEKSKRFRKKLIERWACEIADFFIKNKVGTVQMENLESMKRKEDSYFNIRLRGFWPYAEMQNKIEFKLKQYGIKIRKVAPNNTSKTCSKCGHLNNYFNFEYRKKNKFPHFKCERCSFKENADYNAALNISNPKLKSTKEEP

SEQ ID NO: 2364 - protein, 726 aa, synthetic construct
SEVEFSHEYWMRHALTLAKRARDEREVPVGAILVLNNRVIGEGWNRAIGLHDPTAHAEIMALRQGGLVMQNYRLIDATLYVTFEPCVMCAGAMIHSRIGRVVFGVRNSKHGAAGSLMNVLNYPGMNHRVEITEGILADECAALLCDFYRMPHQVFSARKKAQSSINPGGSSGGSSGSKTPGTSESATPESSGGSSGGSAKNSTTKTLKLRIVRPYNSAEVEKIVADEKNNREKIALEKNKGKVKEACSEHLKVAAYCTTQVERSACLFCKARKLDDRFYQKLRGQFPDAVFWQEISEIFRQLQKQAAEIYNQSLIELYYEILIKGKGIANASRVEHYLSDVCYTRAAELFKNAAIASGLRSKIKSNFRLKELRNMKSGLPTTKSDNFPIPLVKQKGGQCTGFEINNHNSDFIIKIPFGRWQAKKEIDKYRPWEKFDFEQVRKSPKPISLLLSTQRRRRNKGWSRDEGTEAEIRKVMNGDYQASYIEVKRGSKIGEKSAWMLNLSIDVPKIDKGVDPSIIGGIDVGVKSPLVCAINNAFSRYSISDNDLFHFNKKVFARRRILLKKNRHKRAGHGAKNKLKPITILTEKSKRFRKKLIERWACEIADFFIKNKVGTVQMENLESMKRKEDSYFNIRLRGFWPYAEMQNKIEFKLKQYGIEIRKVAPNNTSKTCSKCGHLNNYFNFEYRKKNKFPHFKCEKCNFKENADYNAALNISNPKLKSTKEEP

SEQ ID NO: 2365 - protein, 726 aa, synthetic construct
SEVEFSHEYWMRHALTLAKRARDEREVPVGAILVLNNRVIGEGWNRAIGLHDPTAHAEIMALRQGGLVMQNYRLIDATLYVTFEPCVMCAGAMIHSRIGRVVFGIRNNKHGAAGSLVNVLNYPGMNHRVEITEGILADECAALLCDFYRMPRQVFNARKKAQSSINSGGSSGGGSGSETPSTSESTTPESSGGSSGGPAKNTITKTLKLRIVRPYNSAEVEKIVADEKNNREKTALEKNKDKVKEACSKHLKVAVYCTTQVERNACLFCKARKLDDKFYQKLRGQFPDAVFWQEIGEIFRQLQKQAAEIYNQSLIELYYEIFIKGRGFANASSVEHYLSDVCYTRAAELFKNAAIASGLRGKVKSNFRLKELKNMKSGLPTTKSDNFPIPLVRQKGGQYTGFEISNHDGDFIIKIPFGRWQVKKEINKHRPWEKFDFEQVRKSPKPISLLLSTQRRKRNKGWSKDEGTEAEIRKVMNGDYQTSYIEVKRGSKIGEKSAWMLNLSIDVPKIDKGVDPSIIGGIDVGVKSPLVCAINNALSRYSISDNDLFHFNKKMFARRRILLRKNRHKRAGHGAKNKLKPITMMTEKSKRFRKKLIERWACEIADFFIKNKVGTVQMENLESMKRKEDSYFNIRLRGFWPYAEMQNKIEFKLKQYGIVVRKVAPNNTSKTCSKCGHLNNYFNFEYRKKNKFPHFKCEKCNSKEDADYNAALNISNPKLKSTKGEP

SEQ ID NO: 2366 - protein, 726 aa, synthetic construct
SEVEFSHEYWMRHALTLAKRARDEREVPVGAVLVLNNRIIGEGWNRAIGLHDPTAHAEIMALRQGGLVMQNYRLTDATLYVTFEPCVMCAGAMVHSRIGRVVFGVRNSKRGAAGSLMNVLNYPGVNHCVEITEGILVDECAALLCDFYRMPRQVLNAQKKAQSSISSGGSSGGCSGSETPGASESVTPKSSGGSSAGSTKNTITKTLKLRIVRPYNSAEVEKIVADEKNSREKIALERNKDKVKEACSEHLKVAAYCTTQVERNACLFCKARKLDDRFYQKLRGQFPDAVFWQEIGEIFRQLQKQAAEIYNQSLIELYYEIFIKGKGFANASSMEHYLSDVCYTRAAELFKNAAIASGLRGKVKSNFRLKELKNMRSGLPTAKSDNFPIPLVKQKGGQYTGFEISSHNDDFIIKIPFGRWQVKKEIDKYRPWEKFDFEQVRKSPKPISLLLSTQRRKRNKGWSKDEGTEAEIRKVLNGDYQTSYIEVKRGSKVGEKSAWMLNLSIDVPRIDKGVDPSIIGGIDVGVKSPLVCAINNAFSRYSISDNDLFHFNKKMFARRRILLKKNRRRRAGHGAKNKLKPITILTEKSGRFRKKLIERWACEIADFFVKNKVGTVQMENLESMKRKEDSYFNIRLRGFWPYAEMQNKIEFKLKQYGIKVRKVAPNNTSKTCSKCGHLNNYFSFEYRKKNKFPHFKCEKCNFKENADYNAALNISNPKLKSTKEEL

SEQ ID NO: 2367 - protein, 726 aa, synthetic construct
SEDEFSHEYWMRRALTLAKRARDGREVPVGAVLVLNNRVIGEGWNRAIGLHDPTAHAEIMALRQGGLVMQNYRLIDATLYVTFEPCVMCAGAMVHSRIGRVVFGVRNSKRGAAGSLMNVLDYPGMGHRVEITEGILADECAALLCDFYCMPRQVFNAQKRAQSSINSGGSSGGSSGSETPGTSESATPESSGGGSSGSAKNTITKTLQLRIVRPYNSAEVEKIVADEKNNREKIALEKNKDKVKEACSKHLKVASYCTTQVERNACPFCKARKLDDKFYQKLRGQFPDAVFWQELGEILRQLQKQAAEIYNQSLIELYYEILIKGRGFANASSVEHYLSDVCYTRAAELFKNAAIASGLRGKVKSNFRLKELKNMKSGLPTTKSDNFPIPLVKQKGGQYTGFEISNHNGDFIIKVPFGRWQAKKEIDKYRPWEKFDFEQVRKSPKPISLLLSTQRRKRNRGWSKDEGTEAEIKKVMNGDYQTSYIEVKRGSKIGEKSAWMLNLSIDVPKIDKGVDPSIIGGIDVGVKSPLVCAINNAFSRYSISDNDLFHFNKKMFARRRILLKKSKHKRAGHGAKNKLKPITVLTEKSGRFRKKLIERWACEIADFFIKNRVGTVQMENLESMKRKEDSYFNIRLRGFWPYAEMQNKIEFKLKQYGIEIRKVAPNNTSKTCSRCGHLNNYFNFEYRRKNKFPHFKCEKCNFKENADYNAALNISNPKLKSTKEEP

SEQ ID NO: 2368 - protein, 726 aa, synthetic construct
SEVEYSHEYWMRHALTLAKRARDEREVPVGAILVLNNRVIGVGWNRAIGLHDPTAHAEIMALRQGGLVMQNYRLIDATLYVTFEPCVMCAGAMIHSRIGRVVFGVRNSKHGAAGSLVNVLNYPGMNHRVEITEGILADECAALLCDFYRMPRQVFNARKKAQSSINSGGSSGGSSGSETPGTSESVTPKNSGGSSGSSAKNTITKTLKLRIVRPYNSAEVEKIVADEKNNREKIALEKNKDKVKEACSKHLKVAAYCTTQVERNACLFCKARKLDDKFYQKLRGQFPDAVFWQEIGEIFRQLQKQAAEVYNQSLIELYYEIFIKGKGFANASNVEHYLSDVCYTRAAELFKNAAIASGLRGKVKSNFRLKELKNMKSGLPTTKSDNFPIPLVKQKGGQYTGFEISNHSDDFIIKIPFGRWQVKEEIDKYRPWEKFDFEQVRKNPKPICLLLSTQRRKGNKGWSKDESTEAEIRKVMNGDYQTSYIEVKRGSKIGEKSAWMLNLSIDVPKIDKGVDPSIIGGIDVGVKSPLVCAINNAFSRYSISDNDLFRFNKKMFARRRILLKRNRHKRAGHGAKNKLRPISILTEKSKRFRKKLIERWACEIADFFIKNKVGTVQMESLESLRRKEDSYFNIRLRGFWPYAEMQNKIEFKLKQYGIEIRKVAPNNTSKTCSKCGHLNNYFNFEYRKKNKFPHFKCEKCNFKENADYNAALNISNPKLKSTKEEP

SEQ ID NO: 2369 - protein, 726 aa, synthetic construct
SEVEFSHEYWMRHALTLAKRARDEREVPVGAVLVLNNRVIGVGWNRAIGLHDPTAHAEIMALRQGGLVMQNYRLIDATLYVTFEPCIMCAGAMIHSRIGRVVFGVRNSKRGAAGSLMNVLNYPGMNHRVEITEGILADECAALLCDFYRMPRRVFNARMKAQSSISPGGSSGGSSSSETPGTSESATPESSGGSSGGSAKNTITKTLKLRIVRPYNSAEVEKIVADEKNNREKIALEKNKDKVKEACSKHLKVASYCTTQVERNACPFCKARKLDDKFYQKLRGQFPDAVFWQELGEIFRQLQKQAAEIYNQSLIELYYVIFIKDKGLANASSVEHYLSDVCYTRAAELFKNAAIASGLRGKVKSNFKLKELKSMKSGLPSTKSDNFPIPLVKQRGGQYTGFEISSHNDDFIIKIPFGRWQVKKEIDKYRPWEKFDFEQVRKSPKPISLLLSTQRRKRNKGWSKDEGTEAEIRKVMNGDYQTSYIEVKRGSKTGEKSAWMLNLSIDVPKIDKGVDPSIVGGIDVGVKSPLVCAIDNVLSRYSISDNDLFHFNKKVFARRRILLKKNRHKRAGHGTKNKLKPITILTEKSGRFRKKLIERWACEIANFFIMNKVGTVQMENLESMKRREDCYFNIRLRGFWPYAEMQNKIEFKLKQYGIKIRKVAPNNTSKTCSKCGHLNNYFNFEYRKKNKFPHFKCEKCNFREDADYNAALNISNPKLKSTKEEP

SEQ ID NO: 2370 - protein, 726 aa, synthetic construct; identical to SEQ ID NO: 684

SEQ ID NO: 2371 - protein, 726 aa, synthetic construct
SEVEFSHEYWMRHALTLAERARDAREVPVGAILVLNNRVIGEGWNRAIGQHDPTAHAEIMALRQGGLVMQNYRLIDATLYVTFEPCVMCAGAMIHSRIGRVVFGVRNSKHGAAGSLMNVLNYPGMNHRVEITEGILADECAALLCDFYRMPRQVFNGRKKAQSSINSGGSSGGSSGSETPGTSESATPESSGGSSSGSTKNTITKTLKLRIVRPYNSTEVEKIVADEKNNREKIALEKNKDKVKEACSRHLKVAAYCTTQVERNACLFCKARKLDDKFYQKLRGQFPDAVFWQEISEIFRQLQKQAAEIYNQSLIELYYEILIRGKGIANASRVEHYLSDVCYTRAAELFKNAAIASGLRSKIKSNFRLKELRSMKSGLPTTKSDNFPIPLVRQKGGQYTGFEISNHNSDFIIKIPFGRWQAKKEIDKYRPWEKFDFEQVRKSPKPISLLLSTQRRKRNRGWSKDESTEAEIKKVMNGDYQTSYIEVKRGSKVGEKSAWMLNLSIDVPKIDKGVDPSIIGGIDVGVKSPLVCAINNAFSRYSISDNDLYRFNKKMFARRRILLKKNRHKRAGHGAKNKLRPISILTEKSERFRKKLIERWACEIADFFIRNKVGTVQMENLEGMRRKEDSYFNIRLRGFWPYAEMQNKIEFKLKQYGIEVRKVAPNNTSKTCSKCGHLNNYFNFEYRKKNKFPHFKCEKCNFKENADYNAALNISNPKLKSAKGEP

SEQ ID NO: 2372 - protein, 726 aa, synthetic construct
SEVEFSHEYWMRRALTLAKRARDEREVPVGAVLVLNNRVIGVGWNRAVGLHDPTAHAEIMALRQGGLVMQNYRLIDATLYVTFEPCVMCAGAMIHSRIGRVVFGVRNNKHGAAGSLVNVLDYPGMNHRVEITEGILADECAALLCDFYRMPRQVFNARKKAQSSISPGGSSGGSSGSETPGTSESVTPESSGGSSGGSAKNTITKTLKLRIVRPYNSAEVEKIVADEKNNREKIALEKNKDKVKEACSKHLKVAAYCTTQVERNACLFCKARKLDDKFYQKLRGQFPDAVFWQEIGEVFRQLQKQAAEIYNQSLIELYYEIFIKGKGFANASSVEHYLSDVCYTRAAELFKNAAIASGLRGKVKSNFRLKELKNMKSGLPTTKSDNFPIPLVKQKGGQYTGFEISSHHDDFIIKIPFGRWQVKKEIDKYRPWEKFDFEQVRKSPKPISLLLSIQRRKRNKGWSRDEGTEAEIRKVMNGDYQTSYIEVKRGSKIGEKSAWMLNLSIDVPRIDKGVDPSIIGGIDVGVKSPLVCAINNAFSRYSISDNDLFRFNKKVFARRRILLKKNRHKRAGHGTKNKLKPITILTERSGRFRKKLIERWACEIANFFIKNKVGTVQMENLESMKRKEDSYFNIRLRGFWPYAEMQNKIEFKLKQYGIKIRKVAPNNTSKTCSKCGHLNNYFSFEYRKKSKFPHFRCEKCNFKEDADYNAALNISNPKLKSTKEEP

SEQ ID NO: 2373 - protein, 726 aa, synthetic construct
SEVEFSHEYWMRHALTLAKRARDEREVPVGAVLVLNNRVIGEGWNRTTGLHDPTAHAEIMALRQGGLVMRNYRLTDATLYVTFEPCVMCAGAMIHSRIGRVVFGVRNSKRGAAGSLMNVLNYPGMNHRVEITEGILVDECAALLCDFYRMPRQVLNAQKKAQSSISSGGSPGGCSGSEMPGASESVTPKSSGGSSAGSTKNTITKTLKLRIVRPYNSAEVEKIVADEKNSREKIALERNKDKVKEACSEHLKVAAYCTTQVERSACLFCKARKLDDKFYQKLRGQFPDAVFWQEIGEIFRQLQKQAAEIYNQSLIELYYEIFIKGKGSANASSVEHYLSDVCYTRAAEQFKNAAIASGLRGKVKSNFRLKELKNMKSGLPTTKSDNFPIPLVKQKGGQYTGFEISSHSDDFIIKIPFGRWQVKKEIDKYRPWEKFDFEQVRKSPKPISLLLSTQRRKRNKGWSKDEGTEAEIRKVMNGDYQTSYIEVKRGSKTGEKSAWMLNLSIDVPKIDKGVDPSIIGGIDVGVKSPLVCAINNAFSRYSISDNDLFRFNKKMFARRRILLKKNRHKRAGHGAKNKLKPISILTGKSGRFRKKLIERWACEIADFFIKNKVGTVQMENLESMKRREDSYFNIRLRGFWPYAEMQNKIEFKLKQYGIEIRKVAPDNTSKTCSKCGHLNNYFNFEYRKKNKFPHFKCEKCNFKEDADYNAALNISNPRLKSTKEEP

SEQ ID NO: 2374 - protein, 726 aa, synthetic construct; identical to SEQ ID NO: 684

SEQ ID NO: 2375 - protein, 726 aa, synthetic construct; identical to SEQ ID NO: 684

SEQ ID NO: 2376 - protein, 726 aa, synthetic construct
SEVEFSHEYWMRHALTLAKRARDEREVPVGAILVLNNRVIGEGWNRAIGLHDPTAHAEIMALRQGGLVMQNYRLIDATLYVTFEPCVMCAGAMIHSRIGRVVFGVRNNKHGAAGSLVNVLNYPGMNHRVEITEGILADECAALLCDFYRMPRRVFNAQKKAQSSINSGGSSGGGSSSDTPSTSESTTPEGSGGSSASSTKNTITKTLKLRIVRPYNSAEVEKIVADEKNNREKIALEKNKDKVKEACSEHLRVAAYCTTQVERNACLFCKARKLDDRFYQKLRGQFPDAVFWQEIGEIFRQLQKQAAEIYNQSLIELYYEVFIKGKGFAIASSVEHYLSDVCYTRAAELFKNAAIASGLRGKVKGNFRLKELKNMKSGLPTTKSDNFPIPLVKQKGGQYTGFEISSHNDDFIIKIPFGRWQAKKEIDKYRPWEKFDFEQVRKSPKPISLLLSTQRRKRNKGWSKDEGTEAEIRKVMNGDYQTSYIEVKRGSKIGEKSAWMLNLSIDVPKIDKGVDPSIIGGIDVGVKSPLVCAINNAFSRYSISDNDLFHFNKKMFARRRILLKKNRHKRAGHGAKNKLKPISILTEKSKRFRKKLIERWACEIADFFIKNKVGTVQMENLESMKRKEDSYFNIRLRGFWPYAEMQNKIEFKLKQYGIEIRRVAPSNTSKTCSKCGHLNNYFNFEYRKKNKFPHFKCEKCNFKENADYNAALNISNPKLKSTKEEP

SEQ ID NO: 2377 - protein, 726 aa, synthetic construct
SEVEFSHEYWMRRALTLAKRARDEREVPVGAVLVLNNRVIGEGWNRAIGLHDPTAHAEIMALRQGGLVMQNYRLIDATLYVTFEPCVMCAGAMIHSRIGRVVFGVRNSKHGAAGSLVNVLNYPGMNHCVEITEGILVDECAALLCDFYRMPRQVLNAQKKAQSSISPGGSSGGSSGSETPGASESVTPKSSGGSSGGSAKNTITKTLKLRIVRPYNSAEVEKIVADEKNNREKIALEKNKGKVKEACSKHLEVAAYCTTQVERNACLFCKARKLDDKFYQKLRGQFPDAVFWQEIGEIFRQLQKQAAEIYNQSLIELYYEIFIKGKGFANASSVEHYLSDVCYTRAAELFKNAAIASGLRGKVKSNFRLKELKNMKSGLPTTKSDNFPIPLVKQKGGQYTGFEISSHNDDFIIKIPFGRWQVKKEIDKYRPWEKFDFEQVRKSPKPISLLLSTQRRKRNKGWSKDEGTEAEIRKVMNGDYQTSYIEVKRGSRIGEKSAWMLNLSIDVPKIDKGVDPSIIGGIDVGVKSPLVCAINNAFSRYSINDNDLFRFNKKMFARRRILLKKNRHKRAGHGAKNKLKPFSILTGKSERFRKKLIERWACEIADFFIKNKVGTVQMENLESMKRKEDSYFNIRLRGFWPYAEMQNRIEFKLKQYGIEIRKVAPNNTSKTCSKCGHLNNYFNFEYRRKNKFPHFKCEKCNFKENADYNAALNISNPKLKSTKEEP

SEQ ID NO: 2378 - protein, 726 aa, synthetic construct
SEVEFSHEYWMRHALTLAKRARDEREVPVGAVLVLNNRVIGEGWNRAIGLNDPTVHAEIMALRQGGLVMQNHRLIDATLYVTFEPCVMCAGAMIHSRIGRVVFGVRNSKRGAAGSLMNVLNYPGMNHRVEVTEGILADECAALLCDFYRMPRQVFNAQKKARSNINSGGSSGDSSGSETPGTSESASPESSGGSSGGSAKNTITKTLQLRIVRPYNSAEVEKIVADEKNNREKIALEKNKDKVKEACGKHLKVASYCTTQVERNACLFCKARKLDDKFYQKLRGQFPDAVFWQELGEIFRQLQKQAAEIYNQSLIELYYEIFIKGKGFANASSVEHYLSDVCYTRAAELFKNAAIASGLRGKVKSNFRLKELRNMKSGLPTTKSDNFPIPLVRQKGGQYTGFEISSRNDDFIIKIPFGRWQVKKEIDKYRHWEKFDFEQVRKSPKPISLLLSTQRRKRNKGWSKDEGTEAEIRKVMNGDYRTSYIEVKRGSKTGEKSAWMLNLSIDVPKIDKGVDPSIIGGIDVGVKSPLVCAINNAFGRYSISDNDLFHFNKKMFARRRILLKRNRHKRAGHGAKNKLKPITILTEKSKRFRRKLIERWACEIADFFIKNKVGTVQMENLESMKRKEDSYFNIRLRGFWPYAEMQDKIEFKLKQYGIEIRKVAPNNTSKTCSRCGHLNNYFNFEYRRKNKFPHFKCEKCNFKEDADYNAALNISNPKLKSTKEEP

SEQ ID NO: 2379 - protein, 726 aa, synthetic construct
SEVEFSHEYWMRHALTLAKRARDEREVPVGAVLVLNNRVIGEGWNRAIGLHDPTAHAEIMALRQGGLVMQNYRLIDATLYVTFEPCVMCAGAMIHSRIGRVVFGVRNSKHGAAGSLMNVLDYPGMGHRVEITEGILADECAALLCDFYCMPRQVFNAQKRAQSSINSGGSSGGSSGSETPGTSESATPESSSGGSSGSAKNTITKTLQLRIVRPYNSAEVEKIVADEKNNREKIALEKNKDKVKEACSKHLKVASYCTTQVERNACPFCKARKLDDKFYQKLRGQFPDAVFWQELGEILRQLQKQAAEIYNQSLIELYYEIFIKGKGIANASSVEHYLSDVCYTRAAELFKNAAIASGLRNKVKSNFRLKELRSMKSGLPTTKSDNFPIPLVRQKGGQYTGFEISNHNSDFTIKIPFGRWQAKKEIDKYRPWEKFDFEQVRKSPKPISLLLSTQRRKRNKGWSKDEGTEVEIRKVMNGDYRTSYIEVKRGSKIGEKSAWMLSLSIDVPKIDKGVDPRIIGGIDVGVKSPLVCAINNVLSRYSISDNDLFHFNKKMFARRRILLKKNGHKRAGHGAKNKLKPITIMTEKSKRFRKKLIERWACEIADFFIKNKVGTVQMENLESMKRKEDSYFNIRLRGFWPYAEMQNKIEFKLKQYGIVVRKVAPNNTSKTCSQCGHLNNYFNFEYRKKNKFPYFKCEKCNFKENADYNAALNISNPKLKSTKGEP

SEQ ID NO: 2380 - protein, 726 aa, synthetic construct; identical to SEQ ID NO: 684

SEQ ID NO: 2381 - protein, 726 aa, synthetic construct
SEDEFSHEYWMRHALTLAKRARDGREVPVGAVLVLNNRVIGEGWNRTTGLHDPTAHAEIMALRQGGLVMRNYRLTDATLYVTFEPCVMCAGAMIHSRIGRVVFGVRNSKRGAAGSLMNVLNYPGMNHCVEITEGILVDECAALLCDFYRMPRQVLNAQKKAQSSTNSGGSSGGSSGSETQGTSESATPGSSGGSSGGSAKNTITKTLKLRIVRPYNSAEVEKIVADEKNNREKIALEKNKDKVKEACSKHLKVAAYCTTQVERNACLFCKARKLDDKFYQKLRGQFPDAVFWQEIGEVFRQLQKQAAEIYNQSLIELYYEIFIKGKGFANASSVEHYLSDVCYTRAAELFKNAAIASGLRGKVKSNFRLKELKNMKSGLPTTKSDNFPIPLVKQKGGQYTGFEISSHNDDFIIKIPFGRWQVKKEIDKYRPWEKFDFEQVRKSPKPISLLLSTQRRKRNKGWSKDEGTEAEIRKVMNGDYQTSYIEVKRGSKIGEKNAWTLNLSVDVPKIDKGVDPSIIGGIDVGVKSPLVCAINNALSRYSISDNDLFHFNKKMFARRRILLRKNRHKRAGHGTKNKLRPITILAEKSERFRKKLIERWACEIANFFIKNKVGTVQMENLESMKRKGDSYFNIRLRGFWPYAEMQNKIEFKLKQYGIKIRKVAPNNTSKTCSKCGHLNNYFSFEYRKKNKFPHFKCEKCNFKEDADYNAALNISNPRLKSTKEEP

SEQ ID NO: 2382 - protein, 726 aa, synthetic construct
SEVESSHEYWMRHALTLAKRARDEREVPVGAVLVLNNRVIGEGWNRAIGLHDPTAHAEIMALRRGGLVMQNYRLTDATLYVTFEPCVMCAGAMVHSRIGRVVFGVRNSKRGAAGSLMNVLDYPGMGHRVEITEGILADECAALLCDFYCMPRQVFNAQKRAQSSINSGGSSDGSSGSETPGTSESATPESSGGGSSGSARNTITKTLQLRIVRPYNSAEVEKIVADEKNNREKIALEKNKGKVREACNKHLKVASYCTTQVERNACPFCKARKLDDKFYQKLRGQFPDAVFWQELGEILRQLQKQAAEIYNQSLIELYYEIFIKGKGFANASGVEHYLSDVCYTRAAELFKNAAIASGLRGKVKSNFRLKELKNMRSGLPTTKSDNFPIPLVKQKGGQYAGFEISSHNDDFIIKIPFGRWQVKKEIDKYRPWEKFDFEQVRKSPKPISLLLSTRRRKRNKGWSKDEGTEAEIRKVMNGDYQTSYIEVKRGSKIGEKSAWMLNLSIDVPKIDKGVDPSIIGGIDVGVKSPLVCAINNAFGRYSISDNDLFHFNKKMFAMRRILLKKNRHKRAGHGAKNKLKPITILTEKSKRFRKKLIERWACEIADFFIKNKVGTVQMESLESMKRREDSYFNVRLRGFWPYAEMQNKIEFKLKQYGIEIRKVAPNNTSKTCSKCGHLNNYFNFEYRKKNKFPHFKCEKCNFKENADYNAALNISNPKLKSTKEEP

SEQ ID NO: 2383 - protein, 726 aa, synthetic construct
SEVEFSHEYWMRHALTLAERARDEREVPVGAILVLNNRVIGEGWNRAIGLHDPTAHAEIMALRQGGLVTQNYRLIDATLYVTFEPCVMCAGAMIHSRIGRVVFGVRNNKHGAAGSLVNVLDYPGMNHRVEITEGILADECAALLCDFYRMPRQVFNARKKAQSSISPGGSSGGSSGSETPGTSVSATPESSGGSSGGSAKNTITKTLQLRIVRPYNSAEVEKIVTDEKNNREKIALEKNKDKVKEACSKHLKVASYCTTQVERNACLFCKARKLDDKFYQKLRGQFPDAVFWQELGEIFRQLQKQAAEIYNQSLIELYYEIFIKGKGFANASSVEHYLSDVCYTRAAELFKNAAIASGLRGKVKSNFRLKELKNMKSGLPTTKSDNFPIPLVKQKGGQYTGFEISSHNDDFIIKIPFGRWQVKKEIDKYRPWEKFDFEQVRKSPKPISLLLSTQRRKRNKGWSKDEGTEAEIRKVMNGDYQTSYIEVKRGSKIGEKSAWMLSLSIDVPKIDKGVDPSIIGGIDVGVKSPLVCAIDNAFCRYSISDNDLFHFNKKMFARRRILLKKSRHKRAGHGAKNKLKPISILTEKSKRFRKKLIERWACEIADFFIKNKVGTVQMENLESMKRKEDSYFNIRLRGFWPYAEMQNKIEFKLKQYGIEIRKVAPNNTSKTCSKCGHLNNYFNFEYRKKNKFPHFKCEKCSFKENADYNAALNISNPKLKSTKEEP

SEQ ID NO: 2384 - protein, 726 aa, synthetic construct; identical to SEQ ID NO: 684

SEQ ID NO: 2385 - protein, 726 aa, synthetic construct
SEVEFSHEYWMRHALTLAKRARDEREVPVGAVLVLNNRVIGEGWNRAIGLHDPTAHAEIMALRQGGLVMQNYRLVDATLYVTFEPCVMCAGAMIHSRIGRVVFGVRNSKRGAAGSLMNVLNYPGMNHCVEITEGILVDECAALLCDFYRMPCQVLNARKKAQSGISSGGSSGGSGCSETPGASESVTPKSSGSSSAGSTKNTITKTLKLRIVRPYNSAEVEKIVADEKNNREKIALEKNKDKVQEACSKHLKVASYCTTQVERNACLFCKARKLDDKFYQKLRGQFPDAVFWQELGEIFRQLQKQAAEIYNQSLIELYYKIFIKGKGLANASNVEHYLSDVCYTRAAELFKNAAIASGLRGKVKSNFKLKELKSMKSGLPTTKSDNFPIPLVKQKGGQYTGFEISSHNDDFIIKIPFGRWQVKKEIDKYRPWEKFDFEQVRKSPKPISLLLSTQRRKRNKGWSKDEGTEAEIRKVMNGDYQTSYIEVKRGSKIGEKSAWMLNLSIDVPKIDKGVDPSIIGGIDVGVKSPLVCAINNAFSRYSISDNDLFHYNKRMFARRRILLKKNRHKRAGHGAKNKLKPISILTEKSKRFRKKLIERWACEIADFFIKNKVGTVQMENLESMKRKEDSYFNIRLRGFWPYAEMQNKIEFKLRQYGIVVRKVAPNNTSKTCSKCGHLNNYFNFEYRKKNKFPHFKCEKCNFKEDADYNAALNISNPKLKSTRGEP

SEQ ID NO: 2386 - protein, 726 aa, synthetic construct
SEVEFSHEYWMRHALTLAKRARDEREVPVGAVLVLNNRVIGEGWNRAIGLHDPTAHAEIMALRQGGLVMQNYRLTDATLYVTFEPCVMCAGAMIHSRIGRVVFGVRNSKRGAAGSLMNVLNYPGMNHCVEITEGILVDECAALLCDFYRMPRQVLNAQKKAQSSTNPGGSSGGSSGSETPGTSESATPESSGGSSGGSAKNTITKTLKLRIVRPYNSAEVEKIVADEKNNREKIALEKNKDKVKEACSEHLKVAAYCTSQVERNACLFCKARKLDDKFYQKLRGQFPGAVFWQEIGEIFRQLQKQAAEVYNQSLIELYYEIFIKGKGFANASSVEHYLSDVCYTRAAELFKNAAIASGLRGKVKSNFRLKELKSMKSGLPTTKSDNFPIPLVKQKGGQYTGFEISSHNDDFIIKIPFGRWQVKKEIDKYRPWEKFDFEQVRKSPKPISLLLSTQRRKRNKGWSKDEGTEAEIRKVMNGDYQTSYIEVKRGSKIGEKSAWMLSLSIDVPKIDKGVDPSIIGGIDVGVKSPLVCAINNAFNRYSISDNNLFHFNKKMFARRRILLKKNRHKRAGHGAKNKLKPISILTEKSERFRKKLIERWACEIADFFIRNKVGTVQMENLEGMKRKEDSYFNIRLRGFWPYAEMQNKIEFKLKQYGIEVRKVAPNNTSKTCSKCGHLNNYFNFEYRKKNKFPHFKCEKCNFKENADYNAALNISNPKLKSTKEEP

SEQ ID NO: 2387 - protein, 726 aa, synthetic construct
SEVEFSHEYWMRHALTLAKRARDEREVPVGAILVLNNRVIGEGWNRAIGLHDPTAHAEIMALRQGGLVMQNYRLTDATLYATFEPCVMCAGAMIHSRIGRVVFGVRNSKHGAAGSLVNVLNYPGMNHRVEITEGILADECAGLLCDFYRMPRQVFSARKKAQSSINSGGSSGGSSGSETLGTSESATPEGSGDGSGGSAKNTITKTLKLRIVRPYNSAEVEKIVADEKNNREKIALEKNKGKVKEACSKHLKVAAYCTTQVERNACLFCKARKLDDKFYQKLRGQFPDAVFWQEVGEIFRQLQKQAAEIYNQSLIELYYEIFIKGKGFANASSVEHYLSDVCYTRAAELFKNAAIASGLRGKVKSNFRLKELKNMKSGLPTTKSDNFPIPLVKQKGGQYTGFEISNHNGDFIIKIPFGRWQVKKEINRYRPWEKFDFEQVRKSPKPISLLLSTQRRKKNKGWSKDEGTEAEIRRVMNGDYQTSYIEVKRGSKIGEKSAWMLNLSVDVPKIDKGVDPSIIGGIDVGVKSPLVCAINNALSRYSISDNDLFHFNKRMFARRRILLRGNRHRRAGHGVKNKLKPITILAEKSKRFRKKLIERWACEIANFFIKNKVGTVQMENLESMKRREDSYFNIRLRGFWPYAEMQSKIEFKLKQYGIEVRKVAPNNTSKTCSKCGHLNNYFNFEFRKKNKFPHFKCEKCNFKEDADYNAALNISNPKLKSTKEVP

SEQ ID NO: 2388 - protein, 726 aa, synthetic construct
SEVEFSHEYWMRHALTLAKRARDEREVPVGAILVLNNRVIGGGWNRAIGLHDPTAHAEIMALRQGGLVTQNYRLIDATLYVTFEPCVMCAGAMIHSRIGRVVFGVRNSKHGAAGSLVNVLNYPGMNHRVEITEGILADECAALLCDFYRMPRQVFNARKKAQSSINSGGSSGGSSGSETPGTSESATPESSGGSSGSSAKNTITKTLKLRIVRPYNSAEVEKIVADEKNNREKIALEKNKDKVKEACSKHLKVAAYCTTQVERNACLFCKARKLDDKFYQKLRGQFPDAVFWQEIGEIFRQLQKQAAEIYNQCLIELYYEIFIKGKGFANASSVEHYLSDVCYTRAAELFKNAAIASGLRGKVKSNFRLKELKNMRSGLPTTKSDNFPIPLVKQKGGQYTGFEISSHNDDFIIKIPFGRWQVKKEIDKYRPWERFDFEQVRKNPKPICLLLSTQRRKGNKGWSKDESTEAEIRKVMNGDYQTSYIEVKRGSKIGEKSAWMLNLSIDVPKIDKGVDPSIIGGIDVGVKSPLVCAINNAFSRYSISDNDLFRFNKKVFARRRILLKKNRHKRAGHGTKNKLKPIAILTEKSGRFRKKLIERWACEIANFFIKNKVGTVQMENLESMKRKEDSYFNIRLRGFWPYAEMQNKIEFKLKQYGIKIRKVAPNNTSKTCSKCGHLNNHFSFEYRKKNKFPHFKCEKCNFKEDADYNAALNISNPKLKSTKEEP

SEQ ID NO: 2389 - protein, 726 aa, synthetic construct
SEVEFSHEYWMRHALTLAKRARDEREVPVGAILVLNNRVIGEGWNRAIGLHDPTAHAEIMALRQGGLVMQNYRLIDATLYVTFEPCVMCAGAMIHSRIGRVVFGVRNNKHGAAGSLVNVLDYPGMNHRVEITEGILADECAALLCDFYRMPRQVFNARKKAQSSISPGGSSGGSSGSETPGTSESATPESSGGSSGGSAKNTITKTLKLRIVRPYNSAEVEKIVADEKNNREKTALEKNRDKVKEACSKHLKVAAYCTTQVERNACLFCKARKLDDKFYQKLRGQFPDAVFWQELGEIFRQLQKQAAEIYNQSLIELYYEIFIKGRGFANASSVEHYLSDVCYTRAADLFKNAAIASGLRGKVKGNFRLKELKNMKSGLPTTKSDNFPIPLVKQKGGQYTGFEISSHNDDFIIKVPFGRWQAKKEIDKYRPWEKFDFEQVRKSPKPISLLLSTQRRKRNRGWSKDEGTEAEIRKVMNGDYQTSYIEVKRGSKIGEKSAWMLNLSIDVPKIDKGVEPSIIGGIDVGVKSPLVCAINNAFSRYSISDNDLFRFNKKMFARRRILLGKNRHKRAGHGVKNKLKPITILTEKSGRFRKKLIERWACEIADFFVKNKVGTVQMENLESMKRREDSYFNIRLRGFWPYAEMQNRIEFKLKQYGIEIRKVAPNNTSKTCSKCGHLNNYFNFEFRKKNKFPHFKCEKCNFKENADYNAALNISNPKLKSTKEEP

SEQ ID NO: 2390 - protein, 726 aa, synthetic construct
SEVEFSHEYWMRHALTLAKRARDEREVPVGAILVLNNRVIGEGWNRAIGLHDPTAHAEIMALRQGGLVMQNHRLVDATLYVTFEPCVMCAGAMIHSRIGRVVFGVRNSKRGAAGSLTNVLNYPGMNHRVEITEGILVDECAALLCDFYRMPRQVFNARKKAQSTINSGGSSGGSSGSETPGTSESPTPESSGGSSSGSTKNTITKTLKLRIVRPYNSAEVEKIVADEKNNREKIALEKNKDRVKEACSKHLKVASYCTTQVERNACPFCKARKLDDKFYQKLRDQFPDAVFWQELGEILRQLQKQAAEIYNQSLIELYYEIFIKGRGFANASSVEHYLSDVCYTRAAELFKNAAIASGLRGKVKSNFRLKELKNMKSGLPTTKSDNFPIPLVKQKGGQYTGFEISSRNDDFIIKIPFGRWQVKKEIDKYRPWEKFDFEQVRKSPKPISLLLSTQRRKRNKGWSKDEGTEAEIRKVMNGDYQTSYIEVKRGSKTGEKSAWMLNLSIDVPKIDKGVDPSIIGGIDVGVKSPLICAINNAFSRYGISDNDLFRFNKKVFARRRILLKKNRHKRAGHGTKNKLKPITILTEKSGRFRKKLIERWACEIANFFIKNKVGTVQMEDLESMKRKEDSYFNIRLRGFWPYAEMQNKIEFKLKQYGIEVRKVAPNNTSKTCSKCGHLNNYFGFEYRKKNKFPHFKCEKCNFKEDADYNAALNISNPKLKSTKEEP

SEQ ID NO: 2391 - protein, 726 aa, synthetic construct
SEVEFSHEYWMRHALTLAKRARDEREVPVGAILVLNNRVIGEGWNRAIGLHDPTAHAEIMALRQGGLVMQNYRLIDATLYVTFEPCVMCAGAMIHSRIGRVVFGVRNNKHGAAGSLVNVLNYPGMNHRVEITEGILADECAALLCDFYRMPRQVFNARKKAQSSINPGGSSGGSSGSETPGTSESATPESSGGSSGSSAKNTITKTLKLRIVRPYNSAEVEKIVADEKNNREKIALEKNKDKVKEACSKHLKVASYCTTQVERNACLFCKARKLDDKFYQKLRGQFPDAVFWQELGEIFRQLQKQAAEIYNQSLIELYYEIFIKGKGFANACSVEHYLSDVCYTRAAELFKNAAIASGLRNKIKSNFRLKELKNMKSGLPTTKSDNFPIPLVKQKGGQYTGFEISSHNDDFIIKIPFGRWQVKKEIDKYRPWEKFDFEQVRKSPKPISLLLSTQRRKKNKGWSKDEGTEAEIRKVMNGDYQTSYIEVKRGSRIGEKSAWMLNLSIDVPKIDKGVDPSIIGGIDVGVKSPLVCAINNALSRYSISDNDLFHFNKKMFARRRILLKKNRHRRAGHGAKNKLKPIAVLAEKSEGFRKKLIERWACEVADFFIKNKVGTVQMENLESMKRREDSYFNIRLRGFWPYAEMQNKIEFKLRQYGIEIRKVAPNNTSKTCSKCGHLNNYFDFEYRKKNKFPHFKCEKCNFKENADYNAALNISNPKLKSTKEEP

SEQ ID NO: 2392 - protein, 726 aa, synthetic construct
SEVEFSHEYWMRHALTLAKRARDEREVPVGAILVLNNRVIGEGWNRAIGLHDPTAHAEIMALRQGGLVMQNYRLIDATLYVTFEPCVMCAGALVHSRIGRVVFGVRNSKRGAAGSLMNVLDYPGMGHRVEITEGILADECAALLCDFYCMPRQVFNAQKRAQSGINSGGSSGGSSGSETPGASGSVTPKSSVGSSAGSTKNTITKTLQLRIVRPYNSAEVEKIVADEKNNREKIALEKNKDKVKEACSKHLKVASYCTTQVERNACLFCKARKLDDKFYQKLRGQFPDAVFWQELGEIFRQLQKQAAEIYNQSLIELYYVIFIKGKGLANASSVEHYLSDVCYTRAAELFKNAAIASGLRGKVKSNFKLKELKSMKSGLPSTKSDNFPIPLVKQRGGQYTGFEISSHNDDFIIKIPFGRWQVKKEIDKYRPWEKFDFAQVRKSPKPISLLLSTQRRKRSKGWSKDEGTEAEIRKVMNGDYQTSYIEVKRGSKIGEKSAWMLSLSIDVPKIDKGVDPNIVGGIDVGVKSPLVCAINNALGRFSISDNDLFHFNKKMFARRRILLKKNRHKRAGHGAKNKLKPISILTGKSGRFRKKLIERWACEIADFFIKNKVGTVQMENLESMKRKEDSYFNIRLRGFWPYAEMQNKIEFKLKQYGIKIRKVAPNNTSKTCSKCGHLNNYFNFEYRRKNKFPHFKCEKCNFKENADYNAALNISNPKLKSTKEEP

SEQ ID NO: 2393 - protein, 726 aa, synthetic construct
SEVEFSHEYWMRHALTLAKRARDEREVPVGAILVLNNRVIGEGWNRAIGLHDPTAHAEIMALRQGGLVMQNYRLIDATLYVTFEPCVMCAGAMIHSRIGRVVFGVRNSKRGAAGSLMNVLNYPGMNHRVEITEGILVDECAALLCDFYRMPCQVLNAQKKAQSSISSGGSSGGSSGGDTLGASESVTPKSSVGSSASSTKNTITKTLKLRIVRPYNSAEVEKIVADEKNNREKIALEKNKDKVKEACSKHLKVASYCTTQVERSACPFCKARKLDDKFYQKLRGQFPDAVFWQELGEILRQLQKQAAEVYNQSLIELYYEILIKGKGIANASSVEHYLSDVCYTRAAELFKNAAIASGLRNKIKSNFRLKELRNMKSGLPTTKSDNFPIPLVRQKGGQYTGFEISNHNSDFIIKIPFGRWQAKKEIDKYRPWEKFDFEQVRKSPKPISLLLSTQRRKRNRGWSKDEGTEAEVKKVMNGDYQISYIEVKRGSKIGEKSAWTLNLSIDVPKIDKGVDPSIIGGIDVGVKSPLVCAISNAFSRYSISDNDLFHFNKKMFARRRILLKKSKHKRAGHGVKNKLKPITILTEKSRRFRKKLIERWACEIADFFIKNKVGTVQMENLEGMKRKEDSYFNIRLRGFWPYAEMQNKIEFKLKQYGIEIRKVAPNNTSKTCSKCGHLNNYFNFEYRKKNKFPHFKCEKCSFKENADYNAALNISNPKLKSTKGEP

SEQ ID NO: 2394 - protein, 726 aa, synthetic construct
SEVEFSHEYWMRRALTLAKRARDEREVPVGAVLVLNNRVIGVGWNRAIGLHDPTAHAEIMALRQGGLVMQNYRLTDATLYVTFEPCVMCAGAMIHSRIGRVVFGVRNSKRGAAGSLMNVLNYPGMNHCVEITEGILVDECAALLCDFYRMPRQVLNAQKKAQSSINPGGSSGGSSGSETPGTSESATPESSGGSSGSSAKNTITKTLKLRIVRPYNSAEVEKIVADEKNNREKIALEKNRDKVKEACSKHLKVAAYCTTQVERNACLFCKARKLDDKFYQKLRGQFPDAVFWQEVGEIFRQLQKQAAEIYNRSLIELYYEIFIKGKGFANASSVEHYLSDVCYTRAAELFKNAAIASGLRGKVKSNFRLKELKNMKSGLPTTKSDNFPIPLVKQKGGQYTGFEINSHNDDFIIKIPFGRWQVKKEIDKYRPWEKFDFEQVRKSPKPISLLLSTQRRKRNKGWGKDAGTEAEIRKVMNGDYQTSYIEVKRGSKIGEKSAWMLNLSIDVPKVDKGVDPSIIGGIDVGVKSPLVCAINNAFSRYSISDNDLFRFNKKMFARRRILLKKNRHKRAGHGAKNKLKPISILTEKSERFRKKLIEKWACEIADFFIKNKVGTVQMENLESMKRKEDSYFNIRLRGFWPYAEMQNKIEFKLKQYGIEIRKVAPNNTSKTCSKCGHLNNYFNFEYRKMNKFPHFKCEKCNFKENADYNAALNISNPKLKSTKEEP

SEQ ID NO: 2395 - protein, 725 aa, synthetic construct
SEVEFSHEYWMRHALTLAKRARDEREVPVGAILVLNNRVIGEGWNRAIGLHDPTAHAEIMALRQGGLVMQNYRLIDATLYVTFEPCVMCAGAMIHSRIGRVVFGVRNNKHGAAGSLVNVLNYPGMNHRVEITEGILADECAALLCDFYRMPRQVFNARKKARSNINSGGSSGGSSGSETPGTSESAAPESSGGSSGGSTRNTITKTLKLRIVRPYNSAEVEKIVADEKNNREIALEKNKDKVKEACSKHLKVASYCTTQVERNACPFCKARKLDDKFYQKLRGQFPDAVFWREIGEIFRQLQKQAAEIYNQSLIELYYEIFIKGKGFANASSAEHYLSDVCYTRAAELFKNAAIASGLRGKVKSNFRLKELKNMKSGLPTTKSDNFPIPLVKQKGGKYTGFEISSHSDDFIIKIPFGRWQVKKEIDKYRPWEKFDFEQVRKSPKPISLLLSTQRRKRNKGWSKDEGTEAEIRKVMNGDYQTSYIEVKRGSKIGEKSAWMLNLSIDVPKIDKGVDPSIIGGIDVGVKSPLVCAINNAFSRYSISDNDLFHFNKKMFARRRILLKKNRHKRAGHGAKNKLKPISILTEKSKRFRKKLIERWACEIADFFIKNKVGTVQMENLESMKRKEDSYFNIRLRGFWPYAEMQNKIEFKLKQYGIEIRKVAPNNTSKTCSKCGHLNNYFNFEYRKMNKFPHFKCEKCNFKENADYNAALNISNPKLKSTKEEP

SEQ ID NO: 2396 - protein, 726 aa, synthetic construct
SEVEFSHEYWMRHALTLAKRARDEREVPVGAILVLNNRVIGEGWNRAIGLHDPTAHAEIMAMRQGGLVLQNYRLIDATLYVTFEPCVMCAGAMIHSRIGRVVFGVRNNKHGAAGSLVNVLNYPGMNHRVEITEGILADECAALLCDFYRMPRQVFNAQKRAQSSINSGGSSGGSSGSETQGTSESATPGSSGGGSSGSAKNTITKTLQLRIVRPYNSAEVEKIVADEKNNREKIALEKNKDKVKEACSKHLKVASYCTTQVERNACPFCKARKLDDKFYQKLRGQFPDAVFWQELGEIFRQLQKQAAEIYNQSLIELYYEIFIKGKGITNASRVEHYLSDVCYTRAAELFKNAAIASGLRSKVRSNFRLKELKNMKSGLPTTKSDNFPIPLVKQKGGQYTGFEISSHNDDFIIKIPFGRWQVKKEINKFRPWEKFDFEQVRKSPKPISLLLSTQRRKKNKGWSKDEGTEAEIRRVMNGDYQTSYIEVKRGSKIGEKSAWMLNLSIDVPKIDKGVDPSIIGGIDVGVKSPLVCAINNAFSRYSISDNDLFHFNKKMFARRRILLKKNRHRRAGHGAKNKLKPITILTEKSVRFRKKLIERWACEIADFFIKNKVGTVQMENLESMKRKEDSYFNIRLRGFWPYAEMQNKIGFKLKQYGIKIRKVAPNNTSKTCSKCGHLNNYFSFEYRKKNKFPHFKCEKCNFKEDADYNAALNISNPKLKSTKEEP

SEQ ID NO: 2397 - protein, 726 aa, synthetic construct
SEVEFSHEYWMRHALTLAKRARDEREVPVGAVLVLNNRVIGEGWNRAVGLHDPTAHAEIMALRQGGLVMQNYRLTDATLYATFEPCVMCAGAMIHSRIGRVVFGVRNSKHGAAGSLMNVLNYPGMNHRVEITEGILADECAGLLCDFYRMPRQVFSARKKAQSSIDPGGSSGGSSGGKAPGTSESATLESSGGSSGGSAKNSITKTLKLRIVRPYNSAEVEKIVADEKNNREKIALEKNKGKVKEACSKHLKVATYCTTQVERNACLFCKARKLDDKFYQKLRGQFPDAVFWQEIGEIFRQLQKQAAEIYNQSLIELYYEIFIEGKGSANARSVEHYLSDVCYTRAAELFKNAAIASGLRGKVKGNFRLKELKSMKSGLPTTKSDNFPIPLVKQKGGQYAGFEISSHNDDFIIKIPFGRWQVKKEIDKYRPWEKFDFEQVRKSPKPISLLLSTQRRKRNKGWSKDEGTEAEIRKVMNGDYQTSYIEVKRGSKIGEKSAWMLNLSIDVPKIDKGVDPSIIGGIDVGVKSPLVCAINNAFSRYSISDNDLFRFNKKMFARRRILLKKNRHKRAGHGAKNKLKPITVLTEKSERFRKKLIERWACEIANFFIKNKVGTVQMENLESMKRREDSYFNIRLRGFWPYAEMQNKIEFKLKQYGIEIRKVAPNNTSKTCSKCGHLNNYFSFEFRKKNKFPRFKCEKCSFKENADYNAALNISNPKLKSTKGEP

SEQ ID NO: 2398 - protein, 726 aa, synthetic construct
SEVEFSHEYWMRHALTLAKRARDEREVPVGAVLVLNNRVIGEGWNRAIGLHDPTAHAEIMALRQGGLVMQNYRLTDATLYVTFEPCVMCAGAMIHSRIGRVVFGVRNSKRGAAGSLINVLNYPGMNHCVEITEGILVDECAALLCDFYRMPRQVLNAQKKAQSSVSSGGSSGGGSGSETPGASGSVTPKSSVGNSAGSTKNTITKTLKLRIVRPYNSAEVEKIVADEKSNREKIALEKNRDKVKEACSKHLKVAAYCTTQVERNACLFCKARKLDDKFYQKLRGQFPDAVFWQEIGEIFRQLQKQAAEIYNQSLIELYYEIFIKGKGIANASRVEHYLSDVCYTRAAELFKNAAIASGLRNRIKSNFRLKELKSMKSGLPTTKSDNFPIPLVKQKGGQYAGFEISSHNDDFIIKIPFGRWQVKKEIDKYRPWEKFDFEQVRKSPKPISLLLSTQRRKRNKGWSKDEGTEAEIRKVMNGDYQTSYIEVKRGSKIGEKSAWMLNLSIDVPKIDKGVDPSIIGGIDVGVKSPLVCAINNALSRYSISDNDLFRFNKKMFARRRILLRKNRHKRAGHGARNKLKPITVLTEKSERFRKKLIERWACEIAYFFIKNKVGTVQMENLESMKRREDSYFNIRLRGFWPYAEMQNKIEFKLKQYGIEIRKVAPNNTSKTCSKCGHLNNYFNFEYRKKSKFPHFKCEKCNFKENADYNAALNISNPKLKSTKEEP

SEQ ID NO: 2399 - protein, 726 aa, synthetic construct
SEDEFSHEYWMRHALTLAKRARDGREVPVGAILVLNNRVIGEGWNRAIGLHDPTAHAEIMALRQGGLVMQNYRLTDATLYVTFEPCVMCAGAMIHSRIGRVVFGVRNNKHGAAGSLVNVLNYPGMNHRVEITEGVLADECAALLCDFYRMPRQVFNARKKARSNINSGGSSGGNSGSETPGTSESATPESSGGSPGGSAKNTITKTLKLRIVRPYNSAEVEKIVADEKNNREKIALEKNKDKVKEACSKHLKVAAYCTTQVERNACLFCKARKLDDKFYQKLRGQFPDAVFWQEIGEVFRQLQKQAAEIYNQSLIELYYEIFIKGKGFANASSVEHYLSDVCYTRAAELFKNAAIASGLRGKVKGNFRLKELKNMKSGLPTTKSDNFPIPLVKQKGGQYTGFEISSHNDDFIIKIPFGRWQVKKEIDKYRPWEKFDFEQVRKSPKPISLLLSTQRRKRSKGWSKDEGTEAEIRKVMNGDYQTSYIEVKRGSKIGEKSAWMLNLSIDVPKIDKGVDPSIIGGIDVGVKSPLVCAIDNAFSRYSISDNDLFHFNKKMFARRRILLKKNGHRRAGHGARNKLKPITVLTEKSERFRKKLIERWACEIANFFIKNKVGTVQMENLESMKRREDSYFNIRLRGFWPYAEMQSKIEFKLKQYGIEVRKVAPNNTSKTCSKCGHLNNYFDFEFRKKNKFPHFKCEKCNFKEDADYNAALNISNPKLKSTKEEP

SEQ ID NO: 2400 - protein, 726 aa, synthetic construct; identical to SEQ ID NO: 684

SEQ ID NO: 2401 - protein, 726 aa, synthetic construct
SEVEFSHEYWMRHALTLAKRARDGREVPVGAVLVLNNRVIGEGWNRSIGLHDPTAHAEIMALRQGGLVMQNYRLIDATLYVTFEPCVMCAGAMVHSRIGRVVFGVRNSKRGAAGSLLNVLDHPGMDHRVEITEGILTDECATLLCDFYRMPRQVFNAQKKAQSSTNPSGSSGGSSGSVTPGTSESATPESSGGGFGGSAKNTITKTLQLRIVRPYNSAEVEKIVADEKNNREKIALEKNKDKVKEACSKHLKVASYCTTQVERNACLFCKARKLDDKFYQKLRGQFPDAVFWQELGEIFRQLQKQAAEIYNQSLIELYYEIFIKGKGLANASSVEHYLSDVCYTRAAELFKNAAIASGLRGKVKSNFKLKELKSMKSGLPSTKSDNFPIPLVKQKGGQYTGFEISSHNDDFIIKVPFGRWQVKKEIDKYRPWEKFDFEQVRKSPKPISLLLSTQRRKRNKGWSKDEGTEAEIRKVMNGDYQTSYIEVKRGSKIGEKSAWMLNLSIDVPKIDKGVDPSIIGGIDVGVKSPLVCAINNAFGRYSISDNDLFHFNKKMFARRRILLRKNRHKRAGHGARNKLKPITVLTEKSERFRKKLIERWACEIANFFIKNKVGTVQMENLESMKRREDSYFNIRLRGFWPYAEMQSKIEFRLKQYGIKIRKVAPNNTSKTCSKCGHLNNYFNFEYRKKNKFPHFKCEKCNFKENADYNAALNISNPKLRSTKEEP

SEQ ID NO: 2402 - protein, 726 aa, synthetic construct
SEVEFSHEYWMRHALALAKRARDEREVPVGAVLVLNNRVIGEGWNRAIGQHDPTAHAEIMALRQGGLVMQNYRLTDATLYVTFEPCVMCAGAMIHSRIGRVVFGVRNSKRGAAGSLMNVLNYPGMNHCVEITEGILVDECAALLCDFYRMPRQVLNAQKKAQSSISSGSSSGGSSGSETPGTSESATPESSGGSSGGPAKNTITKTLKLRIVRPYNSAEVEKIVADEKNNREKIALEKNKDKVKEACSKHLKVAAYCTTQVERNACLFCRARKLDDKFYQKLRGQFPDAVFWQELGEILRQLQKQAAEIYNRSLIELYYEIFIKGKGFANASSVEHYLSDVCYTRAAELFKNAAIASGLRSKVRSNFRLKELKNMKSGLPTTKSDNFPIPLVKQKGGQYTGFEISSHNSDFVIKIPFGRWQAKKEIDKYRPWEKFDFEQVRKSPKPISLLLSTQRRKRNKGWSKDEGTEAEIEKVMNGDYQTSYIEVKRGSKTGEKSAWMLNLSIDVPKIDKGVDPCIIGGIDVGVKSPLVCAINDAFSRYSISDNDLFHFNKKMFARRRILLKKSKHKRAGHGAKNKLKPITILTEKSRRFRKKLIERWACEIADFFIKNKVGTVQMENLESMKRREDSYFNIRLRGFWPYAEMQNKIEFKLKQYGIEIRKVAPNNTSKTCSKCGHLNNYFNFEYRKKNKFPHFKCEKCNFKENADYNAALNISNPKLMSTKEEP

SEQ ID NO: 2403 - protein, 726 aa, synthetic construct
SEVEFSHEYWMRHALTLAKRARDEREVPVGAILVLNNRVIGEGWNRAIGLHDPTAHAEIMALRQGGLVMQNYRLIDATLYVTFEPCVMCAGAMIHSRIGRVVFGVRNSKHGAAGSLVNVLNYPGMNHRVGITEGILADECAALLCDFYRMPRQVFNARKKAQSSINPGGSSGGSNGSETPGTSENATPESSGGSSGGSAKSTITKTLKLRIVRPYNSAEVEKIVADEKNNREKIALEKNKDKVKEACSEHLKVAAYCTTQVERSACLFCKARKLDDKFYQKLRGQFPDAVFWQEIGEIFRQLQKQAAGIYNQSLIELYYEIFIKGKGFANASSVEHYLSDVCYTRAAELFKNAAIASGLRGKVKSNFRLKELKNMKSGLPTTKSDNFPIPLVKQKGGQYTGFEISNHNDDFIIKIPFGRWLAKKEIDKYRPWEKFDFEQVRKSPKPISLLLSTQRRKRNKGWSKDEGTEAEIRKVMNGDYQTSYIEVKRGSKIGEKSAWMLNLSIDVPKIDKGVDPSIIGGIDVGVKSPLVCAINNALSRYSISDNDLFHYNKKMFARRRILLKKNRHKRAGHGAKNKLKPISILTEKSKRFRKKLIERWACEIADFFIKNKVGTVQMENLESMKRKEDSYFNIRLRGFWPYAEMQNKIEFKLKQYGIEIRKVAPNNTSKTCSKCGHLNSYFDFEYRKKNKFPHFKCEKCNFKENADYNAALNISNPKLKSTKEEP

SEQ ID NO: 2404 - protein, 726 aa, synthetic construct
SEVEFSHEYWMRHALTLAKRARDEREVPVGAILVLNNRVIGEGWNRAIGLHDPTAHAEIMALRQGGLVMQNYRLIDATLYVTFEPCVMCAGAMIHSRIGRVVFGVRNSKHGAAGSLVNVLNYPGMNHRVEITEGILADECAALLCDFYRMPRQVFNARKKAQSSINPSGSSGGSSGSVTPGTSESATPESSGGGFGGSTKDVITKTLKLRIVRPYNSAEVEKIVADEKNNREKVALEKNKDKVKEACSKHLKVASYCTTQVERNACPFCKARKLDDKFYQKLRGQFPDAVFWQELGEILRQLQKQAAEIYNQSLIELYYEIFIKGRGFANAGSVEHYLSDVCYTRAAELFKNAAIASGLRGKVKSNFRLKELKNMKSGLPTTKSDNFPIPLVKQKGGQYTGFEISSHNDDFIIKIPFGRWQAKKEIDTYRPWEKFDFEQVRKSPKPISLLLSTQRRKRNKGWSKDEGTEAEIRKVMNGDYQTSYIEVKRGSKTGEKSAWMLNLSIDVPKIDKGVDPSIIGGIDVGVKSPLVCAINNAFSRYSISDNDLFRFNKKMFARRRILLKRNRHKRAGHGAKNKLKPITILTEKSVRFRKKLIERWACEIADFFIKNKVGTVQMENLESMKRKEDSYFNIRLRGFWPYAEMQNKIEFKLKQYGIEIRRVAPNNTSRTCSKCGHLNNYFNFEYRRKYKFPHFKCEKCNFKEDADYNAALNISNPKLKSTKEEP

SEQ ID NO: 2405 - protein, 726 aa, synthetic construct
SEDEFSHEYWMRHALTLAKRARDEREVPVGAILVLNNRVIGEGWNRAIGLHDPTAHAEIMALRQGGLVMQNYRLIDATLYVTFEPCVMCAGAMIHSRIGRVVFGVRNSRRGAAGSLMNVLGYPGMNHRVEITEGILADECAALLCDFYRMPRQVFNTQKKAQSGFNSGGSSGCGSGSETPGTSESATPESSGGSSGGSAKSTITKTLKLRIVRPYNSAEVEKIVADEKNNREKIALEKNKDKVKEACSEHLKVATYCTTQVERNACLFCKARKLDDKFYQKLRGQFPDAVFWQELGEIFRQLQKQAAEIYNQSLIELYYEIFIKGKGITNASRVEHYLSDVCYTRAAELFKNAAIASGLRSKVRSNFRLKELKNMKSGLPTTRSDNFPIPLVKQKGGQYAGFEISSHNDDFIIKIPFGRWQAKKEIDKYRPWEKFDFEQVRRSPKPISLLLSTQRRKRNKGWSKDEGTEAEIRKVMNGDYQTSYIEVKRSSKTGEKSAWMLNLSIDVPKIDKGVDPSIIGGIDVGVKSPLVCAINNAFSRYSISDNDLFHFNKKMFARRRILLKKNRHKRAGHGAKNKLKPISILTEKSKRFRKKLIERWACEIADFFIKNKVGTVQMENLESMKRKEDSYFNIRLRGFWPYAEMQNKIEFKLKQYGIEIRKVAPNNTSKTCSKCGHLNNYFNFEYRRKNKFPHFKCEKCNFKEDADYNAALNISNPKLKSTKEEP

SEQ ID NO: 2406 - protein, 726 aa, synthetic construct
SEVEFSHEYWMRHALTLAKRARDEREVPVGAVLVLNNRIIGEGWNRAIGLHDPTAHAEIMALRQGGLVMQNYRLTDATLYVTFEPCVMCAGAMVHGRIGRVVFGVRNSKRGAAGSLMNVLNYPGVNHCVEITEGILVDECAALLCDFYRMPRRVLNAQKKAQSSISPGGSSGGCSGSEMPGASESVTPKSSGGSSAGSTKNTITKTLKLRIVRPYNSAEVEKIVADEKDNREKIALEKNRDKVKEACSKHLKVAAYCTTQVERNACLFCKARKLDDKFYQKLRGQFPDAVFWQEIGEIFRQLQKQAAEIYNQSLIELYYEIFIKGKGFANASSVEHYLSDVCYTRAAELFKNAAIASGLRGKVKSNFRLKELKNMKSGLPTTKSDNFPIPLVKQKGGQYTGFEISSHNDDFIIKIPFGRWQVKKEINKYRPWEKFDFEQVRKNPKPISLLLSIQRRKRNKGWSRDEGTEAEIRKVMNGDYQTSYIEVKRGSKIGEKSTWMLNLSIDVPKIDKGVDPSIIGGIDVGVKSPLICAINNAFSRYGISDNDLFRFNKKVFARRRILLKKNRHKRAGHGTKNKLKPITILTEKSGRFRKKLIERWACEIANFFIKNKVGTVQMENLESMKRKEDSYFNIRLRGLWPYAEMQNKIEFKLKQYGIKIRKVAPNNTSKTCSKCGHLNNYFSFEYRKKNKFPHFKCEKCNFKEDADYNAALNISNPKLKSTKEEP

SEQ ID NO: 2407 - protein, 726 aa, synthetic construct
SEVEFSHEYWMCHALTLAKRARDEREVPVGAVLVLNNRVIGVGWNRAIGLHDPTAHAEIMALRQGGLVLQNYRQTDATLYVTFEPCVMCAGAMIHSRIGRVVFGVRNSKRGAAGSLMNVLNYPGMNHRVEITEGILADECAALLCDFYHMPRQVFNAQKKAQSSINSGGSSGGSSGSETPGTSESATPKSSGGSSGGSAKNTITKALKLRIVRPYNSAEVEKIVADEKNNRERIALEKNKDKVKEACSKHLKVAAYCTTQVERNACLFCRARKLDDKFYQKLRDQFPEAVFWQEIGEIFRQLQKQAAEIYNQSLIELYYEIFIKGKGIANASSVEHYLSDVCYTKAAELFKNAAIASGLRSKIKSNFRLKELRNMKSGLPTTKSDNFPIPLVKQKGGQYTGFEISNHNSDLVIKIPFGRWQVKKEIDKYRPWEKFDFEQVRKSPKPISLLLSTQRRKRNKGWSKDEGTEAEIKKVMNGDYQTSYIEVTRGSKIGEKSAWMLNLSIDVPKIDKGVDPSIIGGIDVGVKSPLVCAINNAFSRYSIGDNDLFHFNKKMFARRRILLKKNRHKRAGHGAKNKLKPITILTEKSKRFRKKLIERWACEIADFFVKNKVGTVQMEDLESMKRKEDSYFNIRLRGFWPYTEMQNKIEFKLKQYGIEIRKVAPNNTSKTCSKCGHLNIYFNFEYRKKNKFPHFKCEKCNFKENADYNAALNICNPKLRSTKEEP

SEQ ID NO: 2408 - protein, 726 aa, synthetic construct
SEVEFNHEYWMRHALTLAKRARDEGEVPVGAILVLNNRVIGVGWNRAIGLHDPTAHAEIMALRQGGLVMQNYRLIDATLYVTFEPCVMCAGAMIHSRIGRVVFGVRNSKHGAAGSLVNVLNYPGMNHRVEITEGILADECAALLCDFYRMPRQVFNARKKAQSSINSGGSSGGSSGSETPGTSESATPKSSGGSSGGSAKNTITKALKLRIVRPYNSAEVEKIVADEKNNRERIALEKNKDKVKEACSKHLKVAAYCTTQVERNACLFCKARKLDDKFYQKLRGQFPDAVFWQEIGEIFRQLQKQAAEIYNQSLIELYYEILIKGKGFANASSVEHYLSDVCYARAAELFKNAAIASGLRGKVKSNFRLKELKNMRSGLPTTKSDNFPIPLVKQKGGQYAGFEISSHNDDFIIKIPFGRWQVKKEIDKYRPWEKFDFEQVRKSPKPISLLLSTRRRKRNKGWSKDEGTEAEIRKVMNGDYQTSYIEVKRGSKIGEKSAWMLNLSIDVPKIDKGVDPSIIGGIDVGVKSPLVCAINNALSRYSISDNDLFHFNKKMFARRRILLRKNRHKRAGHGARNKLKPITVLTEKSERFRKKLIERWACEIANFFIKNKVGTVQMENLESMKRREDSYFNIRLRGFWPYAEMQNKIEFKLKQYGIEIRKVAPNNTSKTCSKCGHLNNYFNFEFRKKNKFPHFKCEKCNFKENADYNAALNISNPKLKSTKEEP

SEQ ID NO: 2409 - protein, 726 aa, synthetic construct
SEVEFSHEYWMRHALTLAKRARDGREVPVGAVLVLNNRVIGEGWNRAIGLHDPTAHAEIMALRQGGLVMQNYRLTDATLYVTFEPCVMCAGAMVHSRIGRVVFGVRNSKRGAAGSLMNVLDYPGMDHRVEITEGILADECAALLCDFYRMPHQVFNAQKKAQSSINSGGSSGGNSGSKTPGTSESATPESSGGSSGGSAKNTITKTLKLRIVRPYNSAEVEKIVADEKNNREKIALEKNKDKVKEACSKHLKVAAYCTTQVERNACQFCKARKLDDKFYQKLRGQFPDAVFWQELGEIFRQLQKQAAEIYNQSLIELYYEIFIKGKGFANASSVEHYLSDVCYTRAAELFKNAAIASGLRGKVKSNFKLKELKSMKSGLPSTKSDNFPIPLVKQKGGQYTGFEISSHNDDFIIKIPFGRWQVKKEIDKYRPWEKFDFEQVRKSPKPISLLLSTQRRKRNKGWSKDEGTEAEIRKVMNGDYRTSYIEVKRGSKTGEKSAWMLNLSIDVPKIDKGVDPSIVGGIDVGVKSPLVCAIDNVHSRYSISDNDLFHFNKKMFARRRILLKKNRHRRAGHGAKNKLKPISILTEKSKRFRKKLIERWACEIADFFIKNKVGTVQMENLESMKRKEDSYFNIRLRGFWPYAEMQNKIEFKLKQYSIKIRKVAPNNTSKTCSKCGHLNNYFSFEYRKKNKFPHFKCEKCNFKENADYNAALNISNPKLMSTKEEP

SEQ ID NO: 2410 - protein, 726 aa, synthetic construct
SEAEFSHEYWMRRALTLAKRARDEREVPVGAVLVLNNRVIGVGWNRAVGLHDPTAHAEIMALRQGGLVMQNYRLVEATLYVTFEPCIMCAGAMIHSRIGRVVFGVRNSKRGAAGSLMNVLNHPGMNHRVEITEGILADECAALLCDYYRMPRQVFNARKKAQPSINSGGSSGGNSGSETPGTSESATPGSSGGGSSGSAKNTITKTLQLRIVRPYNSAEVEKIVADEKNNREKIALEKNKDKVKEACSKHLKVASYCTTQVERNACPFCKARKLDDKFYQKLRGQFPDAVFWQELGEIFRQLQKQAAEIYNQSLIELYYEIFIKGKGITNASRVEHYLSDVCYTRAAELFKNAAIASGLRSKVRSNFRLKELKNMKSGLPTTKSDNFPIPLVKQKGGQYTGFEISSHNDDFIIKIPFGRWQVKKEINKFRPWEKFDFEQVRKSPKPISLLLSIQRRKRSKGWSKDEGTEAEIRKVMNGDYQTSYIEVKRGSKIGEKSAWMLNLSIDVPKIDKGVDPSIIGGIDVGVKSPLVCAINNAFSRYSISDNDLFHFNKKMFARRRILLKKNRHRRAGHGAKNKLKPITILTEKSVRFRKKLIERWACEIADFFIKNKVGTVQMENLESMKRKEDSYFNIRLRGFWPYAEMQNKIGFKLKQYGIKIRKVAPNNTSKTCSKCGHLNNYFSFEYRKKNKFPHFKCEKCNFKEDADYNAALNISNPKLKSTKEEP

SEQ ID NO: 2411 - protein, 726 aa, synthetic construct
SEVEFSHEYWMRHALTLAKRARDEREVPVGAILVLNNRVIGVGWNRAIGLHDPTAHAEIMALRQGGLVTQNYRLINATLYVTFEPCVMCAGAMIHSRIGRVVFGVRNSKHGAAGSLVNVLNYPGMNHRVEITEGILADECAALLCDFYRMPRQVFNARKKAQSSINSGGSSGGSSGSETPGTSESATPKSSGGSSGGSAKNTITKTLKLRIVRPYNSTEVEKIVADEKNNREKIALEKNKDKVKEACSKHLKVASYCTTQVERNACLFCKARKLDDKFYQKLRGQFPDAVFWQELGEIFRQLQKQAAEIYNQSLIELYYEIFIKGKGFANASSVEHYLSDVCYTRAAELFKNAAIASGLRGKVKSNFRLKELKNMKSGLPTTKSDNFPIPLVKQKGGQYTGFEVSSHNDDFIIKIPFGRWQVKKEIDKYRPWEKFDFEQVRKSPRPISLLLSTQRRKRNKGWSKDEGTEAEIRKVMNGDYQTSYIEVKRGSKIGEKSAWMLNLSIDVPKIDKGVDPSIIGGIDVGVKSPLVCAINNAFSRSSISDNELFHFNKKMFARRRILLKKNRYKRAGHGAKNKLKPITIMTEKSKRFRKKLIERWACEIADFFIKNRVGTVQMENLESMKRKEDSYFNIRLRGFWPYAEMQNKIEFKLKQYGIEIRKVAPNNTSKTCSKCGHLNNYFNFEYRKKNKFPHFKCEKCNFKENADYNAALNISNPKLKSTKEEP

SEQ ID NO: 2412 - protein, 726 aa, synthetic construct
SEVEFSHEYWMRHALTLAKRARDECEVPVGAILVLNNRVIGEGWNRAIGLHDPTAHAEIMALRQGGLVMQNYRLIDATLYVTFEPCVMCAGAMVHSRIGRVVFGVRNSKRGAAGSLMNVLDYPGMGHRVEITEGILADECAALLCDFYCMPRRVFNAQKRAQSSINSGGSSGGSSGSETPGTSESATPESSGGGSSGSAKNTITKTLQLRIVRPYNSAEVEKIVTDEKNNREKIALEKNKDKVKEACSKHLKMASYCTTQVERNACLFCRARKLDDKFYQKLRGQFPEAVFWQEIGEIFRQLQKQAAEIYNQSLIELYYEIFIKGKGFANASSVEHYLSDVCYTRAAELFKNAAIASGLRGKVKSNFRLKELKNMKSGLPTTKSDNFPIPLVRQKGGQYTGFEISSHNDDFIIKIPFGRWQVKKEIDKYRPWEKFDFEQVRKSPKPISLLLSTQRRKKNRGWSKDEGTEAEIKKVMNGDYQTSYIEVKRGSKIGEKSAWMLSLSIDVPKIDKGVDPSIIGGIDVGVKSPLVCAISNAFSRYSISDNDLFHFNKKMFARRRILLKKSKHKRAGHGAKNKLKPITILTEKSRRFRKKLIERWACEIADFFIKNKVGTVQMENLESMKRKEDSYFNIRLRGFWPYAEMQNKIEFKLKQYGIEIRKVAPNNTSKTCSKCGHLNNYFNFEYRKKNKFPHFKCEKCNFKENADYNAALNISNPKLKSTKEEP

SEQ ID NO: 2413 - protein, 726 aa, synthetic construct
SEVEFSHEYWMRHALTLAKRARDEREVPVGAVLVLNNRVIGEGWNRAIGLHDPTAHAEIMALRQGGLVMQNYRLVDATLYVTFEPCVLCAGAMVHSRIGRVVFGVRNNKRGAAGSLMNVLDYPGMNHRVEITEGILADECAALLCDFYRMPRQVFNAQKKARPNINSGGSSGGRSGSETPGTSESTTPESSGGSSGGSAKNTITKTLKLRIVRPYNSAEVEKIVADEKNNRERVALEKNKDKVKEACSEHLRVAAYCTTQVERNACLFCKARKLDDKFYQKLRGQFPDAVFWQELGEILRQLQKQAAEIYNQSLIELYYEIFIKGRGFANASSVEHYLSDVCYTRAAELFKNAAIASGLRGKVKSNFRLKELKNMKSGLPTTKSDNFPIPLVKQKGGQYTGFEISSHNDDFIIKIPFGRWQVKKEIDKYRPWEKFDFEQVRKSPKPISLLLSTQSRKRSKGWSKDEGTEAEIRKVMNGDYQTSYIEVKRGSKIGEKSAWTLNLSIDVPKIDKGVDPSIIGGIDVGVKSPLVCAINNALSRYSISDNDLFHFNKKMFARRRILLKKNRHKRAGHGARNKLKPIAVLTEKSKRFRKKLIERWACEIANFFIKNRVGTVQMENLESMKRKEDSYFNIRLRGFWPYAEMQNKIEFKLRQYGIEIRKVAPNNTSKTCSKCGHLNNYFNFEYRKKNKFPYFKCEKCNFKENADYNAALNVSNPKLKSTKEEP

SEQ ID NO: 2414 - protein, 726 aa, synthetic construct
SEDEFSHEYWMRHALTLAKRARDGREVPVGAVLVLNNRVIGEGWNRAIGLHDPTAHAEIMALRQGGLVMQNYRLIDATLYVTFEPCVMCAGAMVHSRIGRVVFGVRNSKRGAAGSLMNVLDYPGMGHRVEITEGILADECAALLCDFYCMPRQVFNAQKRAQSSISSGGSSGGSSGSETPGTCESATPGSSGGSSGGSAKNTITKTLKLRIVRPYNSAEVEKIVADEKNNREKIALEKNKDKVKEACSEHLKVAAYCTTQVERNACLFCKARKLDDKFYQKLRGQFPDAVFWQETGEIFRQLQRQAAEIYNQSLIELYYEIFIKGKGFANASSVEHYLSDVCYTRAAELFKNAAIASGLRGKVKSNFRLKELRNMKSGLPTTKSDNFPIPLVKQKGGQYTGFEISSHNDDFIIKIPFGRWQVKEEIDKYRPWEKFDFEQVRRNPKPISLLLSTQRRKRNKGWSKDEGTEAEIRKVMNGDYQTSYIEVKRGSKIGEKSGWMLNLSIDVPKIDKGVDPRIIGGIDVGVRSPLVCAINNAFSRYSIGDNDLFHYNKKMFARRRILLKKNRHRRAGHGARNKLKPITILTEKSKRFRKKLIERWACEIADFFIKNKVGTVQMENLESMKRKEDSYFNIRLRGFWPYAEMQNKIEFKLKQYGIEIRKVAPNNTSKTCSKCGHLNNYFNFEYRKKNKFPHFKCEKCNFKENADYNAALNISNPKLKSAKEEP

SEQ ID NO: 2415 - protein, 726 aa, synthetic construct
SEVEFSHEYWMRHALTLAKRARDEREVPVGAILVLNNRVIGEGWNRAIGLHDPTAHAEIMALRQGGLVMQNYRLIDATLYVTFEPCVMCAGAMIHSRIGRVVFGVRNNKHGAAGSLVNVLNYPGMNHRVEITEGILADECAALLCDFYRMPRQVFNARKKAQSSINPGGSSGGSSGSGTPGTSESATPESSGGSSGSSAKNTITKTLKLRIVRPYNSAEVEKIVADEKNNREKIALEKNKDKVKEACSKHLKVAAYCTTQVERNACLFCKARRLDDKFYQKLRGQFPDAVFWQEIGEIFRQLQKQAAEIYNQSLVELYYEILIKGKGIANASSVEHYLSDVCYTRAAGLFKNAAIASGLRNKIKSNFRLKELRNMKSGLPTTKSDNFPIPLVKQKGGQYTGFEISNHDGDFIIKIPFGRWQVKREINKHRPWEKFDFEQVRKSPKPISLLLSTQRRKRNKGWSKDEGTEAEIRKVMNGDYQTSYIEVKRGSKIGEKSAWMLNLSIDVPKIDKGVDPSIIGGIDVGVKSPLVCAINNALSRYSISDNDLFHFNKKMFARRRILLRKNRHKRAGHGARNKLKLITVLTEKSERFRKKLIERWACEIANFFIKNKVGTVQMENLESMKRREDSYFNIRLRGFWPYAEMQNKIEFKLKQYGIEVRKVAPNNTSKTCSKCGHLNNYFNFEFRKKNKFPHFKCEKCNFKEDADYNAALNISNPKLKSTKEEP

SEQ ID NO: 2416 - protein, 726 aa, synthetic construct; identical to SEQ ID NO: 684

SEQ ID NO: 2417 - protein, 726 aa, synthetic construct
SEVEFSHEYWMRHALTLAKRARDEREVPVGAVLVLNNRVIGEGWNRAIGLHDPTAHAEIMALRQGGLVMQNYRLIDATLYVTFEPCVMCAGAMVHSRIGRVVFGVRNSKRGAAGSLMNVLDYPGMGHRVEITEGILADECAALLCDFYCMPRQVFNAQKRAQSSINSGGSSGGSSGSETPGTSESATPESSGGGSSGSAKNTITKTLQLRIVRPYNSAEVEKIVADEKNNREKIALEKNKDKVKEACSKHLKVASYCTTQVERNACPFCKARKLDDKFYQELRGQFPDAVFWQELGEILRQLQKQAAEIYNQSLIELYYEIFIKGRGFANAGGVEHYLSDVCYTRAAVLFKNAAIASGLRGKVKSNFRLKELKNMKSGLPTTKSDNFPIPLVKQKGGQYTGFEISSHNDDFIIKIPFGRWQVKKEIDKYRPWEKFDFEQVRKSPKPISLLLSTQRRKRNKGWSKDEGTEAEIRKVMNGDYQTSYIEVKRGSKTGEKSAWMLNLSIDVPKIDKGVDPSIIGGIDVGVKSPLVCAVNNAFSRYSISDNDLFRFNKKMFARRRILLRKNRHKRAGHGAKNKLKPISILTGKSERFRKKLIERWACEIADFFIKNKVGTVQMENLESMKRKEDSYFNIRLRGFWPYAEMQNKIEFKLKQYGIVVRKVAPNNTSKTCSRCGHPNNYFNFEYRKKNKFPHFKCEKCNFKEDADYNAALNISNPKLKSTKEEP

SEQ ID NO: 2418 - protein, 726 aa, synthetic construct
SEVEFSHEYWMRHALTLAKRARDEREVPVGAVLVLNNRVIGEGWNRAIGLHDPTAHAEIMALHQGGLVMQNYRLIDATLYVTFEPCVMCAGAMIHSRIGRVVFGARNSKRGAAGSLMNVLSYPGMNHRVEITEGILADECAALLCDFYRMPRRVFNAQKKAQSSINSGGSSGGGSSSDTPSTSESTTPESSGGSSGGPAKNTITKTLKLRIVRPYNSAEVEKIVADEKNNREKTALEKNKDKVKEACSKHLKVAAYCTTQVERNACLFCKARKLDDKFYQKLRGQFPDAVFWQELGEILRQLQKQAAEIYNQSLIELYYEIFIKGRGFANASSVEHYLSDVCYTRAAELFKNAAIASGLRGKVKSNFRLKELKNMKSGLPTTKSDNFPIPLVKQKGGQYTGFEISSHNDDFIIKIPFGRWQEKEEIDKYRPWEKFDFEQVRRSPKPISLLLSTQRRKKNKGWSKDEGTEAEIRRVMNGDYQTSYIEVKRGSKIGEKGAWMLNLSIDVPKIDKGVDPSIIGGIDVGVKSPLVCAINNAFSRYSICDNDLFRFNKKMFARRRILLKKNRHKRAGHGAKNKLKPISILTEKSERFRKKLIEKWACEIADFFIKNKVGTVQMENLESMKRREDSYFNIRLRGFWPYAEMQNKIEFKLKQYGIEIRKVAPNNTSKTCSKCGHLNNYFNFEYRKKNKFPHFRCEKCNFKENADYNAALNISNPKLKSTKEEP

SEQ ID NO: 2419 - protein, 726 aa, synthetic construct
SEDEFSHEYWMRHALTLAKRARDEREVPVGAILVLNNRVIGEGWNRAIGLHDPTAHAEIMALRQGGLVMQNYRLIDATLYVTFEPCVMCAGAMIHSRIGRVVFGVRNSKHGAAGSLMNVLNYPGMNHRVEITEGILADECAALLCDFYRMPHQVFSARKKAQSSINPGGSSGGSSGSKTPGTSESATPESSGGSSGGSAKNSITKTLKLRIVRPYNSAEVEKIVADEKNNREKIALEKNKGKVKEACSKHLKVATYCTTQVERNACLFCKARKLDDKFYQKLRGQFPDAVFWQEIGEIFRQLQKQAAEIYNQSLIELYYEIFIEGKGFANASSVEHYLSDVCYTRAAELFKNAAIASGLRGKVKGNFRLKELKSMKSGLPTTKSDNFPIPLVKQKGGQYTGFEISSHNDDFIIKIPFGRWQVKKEIDRYRPWEKFDFEQVRKSPKPISLLLSTQRRKRNKGWSKDEGTEAEIRKVMNGDYQTSYIEVKRGSKIGEKSAWMLSLSIDVPKIDKGVNPSIIGGIDVGVRSPLVCAIDNAFSRYSISDNDLFHFNKKMFARRRILLKKNRHKRAGHGAKNKLKPISILTEKSKRFRKKLIERWACEIADFFIKNKVGTVQMENLESMKRKEDSYFNIRLRGLWPYAEMQNKIEFKLKQYGIEIRKVAPNNTSKTCSKCGHLNNYFNFEYRKKNKFPHFKCEKCNFKEDADYNAALNISNPKLKSTKEEP

SEQ ID NO: 2420 - protein, 726 aa, synthetic construct
SEVEFSHEYWMRHALTLAKRARDEREVPVGAVLVLNNRVIGEGWNRAIGLHDPTAHAEIMALRQGGLVMQNYRLVDATLYVTFEPCVLCAGAMVHSRIGRVVFGVRNSKRGAAGSLMNVLNYPGMNHRVEITEGILADECAALLCDFYRMPRQVFNARKKAQSSINPGGSSGGSSGSETPGTSESATPESSGGSSGSSAKNTITKTLKLRIVRPYNSAEVEKIVVDEKNNREKIALEKNKDKVKEACSKHLKVAAYCTTQVERNACLFCKARRLDDKFYQKLRGQFPDAVFWQEIGEIFRQLQKQAAEVYNQSLIELYYEIFIKGKGFANASSVEHYLSDVCYTRAAELFKNAAIASGLRGKVKSNFRLRELKNMKSGLPTTKSDNFPIPLVKQKGGQYTGFEISNHNSDFIIKIPFGRWQVKKEINKYRPWEKFDFEQVRKSPKPISLLLSTQRRKRNKGWSKDEGTEAEIRKVMNGDYQTSYIEVKRGSRIGEKSAWMLSLSIDVPKIDRGVDPSIIGGIDVGVKSPLVCAINNAFSRYSISDNDLFRFNKKMFARRRILLKKNRHKRAGHGAKNKLKPISILTGKSERFRKKLIERWACEIADFFIRNKVGTVQMENLESMKRKEDSYFNIRLRGFWPYAEMQNKIEFKLKQYGIVIRKVAPNNTSKTCSKCGHLNDYFNFEYRKKNKFPHFKCERCNFKENADYNAALNISNPKLKSTKGEP

SEQ ID NO: 2421 - protein, 726 aa, synthetic construct
SEDEFSHEYWMRHALTLAKRARDGREVPVGAVLVLNNRVIGEGWNRAIGLHDPTAHAEIMALRQGGLVMQNYRLIDATLYVTFEPCVMCAGAMVHSRIGRVVFGVRNSKRGAAGSLMNVLDYPGMGHRVEITEGILADECAALLCDFYCMPRQVFNAQKRAQSSINSGGSSGGSSGSETPGTSESVTPKSSGGSSAGSTKDTITKTLKLRIVRPYNSAEVEKVVADEKNNREKIAIEKNKDMVKEACSKHLKVASYCTTQVERNACLFCKARKLDDKFYQKLRGQFPDAVFWQELGGIFRQLQKQAAEIYNQSLIELYYEIFIKGKGITNASRVEHYLSDVCYTRAAELFKNAAIASGLRSKVRSNFRLKELKNMKSGLPTTKSDNFPIPLVKQKGGQYTGFEISSHNSDFIIKIPFGRWQEKEEIDKYRPWEKFDFEQVRRSPKPISLLLSTQRRKKNKGWSKDEGTEAEIRRVMNGDYQTSYIEVKRGSKIGEKSAWMLNLSIDVPKIDKGVDPSIIGGIDVGVKSPLVCAINNAFSRYSISDNDLFHFNKKMFARRRILLKKTRHKRAGHGAKNKLKPISILTEKSERFRKKLIERWACEIADFFIKNKVGTVQMENLESMKRREDSYFNIRLRGFWPYAKMQNKIEFKLKQYGIEIRKVAPNNTSKTCSKCGHLNNYFNFEYRKKNKFPHFKCEKCNFKENADYNAALNISNPKLKSTKEEP

SEQ ID NO: 2422 - protein, 726 aa, synthetic construct
SEVEFSHEYWMRHALTLAKRARDEREVPVGAVLVLNNRVIGEGWNRAIGLHDPTAHAEIMALRQGGLVMQNYRLTDATLYVTFEPCVMCAGAMIHSRIGRVVFGIRNSKRGAAGSLMNVLNYPGMNHCVEITEGILVDECAALLCDFYRMPRQVFNAQKRAQSSISSGGSSGGSSGSGTPGASESVAPKSSVGSSAGSSKNTTTKTLKLRIVRPYNSAEVEKIVADEKNNREKVALEKNKDKVKEACSKHLKVAAYCTTQVERNACLFCKARRLDDKFYQKLRGQFPDAVFWQEIGEIFRQLQKQAAEVYNQSLVELYYEILIKGKGIANASSVEHYLSDVCYTRAAELFKNAAIASGLRNKIKSNFRLKELRNMKSGLPTTKSDNFPIPLVKQKGGQYTGFEISSHNDDFIIKIPFGRWQVKKEIDKYRPWEKFDFEQVRKSPKPISLLLSTQRRKKNKGWSKDEGTEAEIRRVMNGDYQTSYIEVKRGSKIGEKSAWMLNLSIDVPKIDKGVDPSIIGGIDVGVKSPLVCAINNAFSRYSISDNDLFHFNKKMFARRRILLKKNRRRRAGHGAKNKLKPISILTGKSERFRKKLIERWACEIADFFIKNKVGTVQMENLENIKRKEDSYFNIRLRGFWPYAEMQNKIEFKLKQYGIEVRKVAPNNTSKTCSKCGHLNNYFNFEYRKKNKFPHFKCEKCNFKEDADYNAALNISNPKLKSTKEEP

SEQ ID NO: 2423 - protein, 726 aa, synthetic construct
SEVEFSHEYWMRHALTLAKRARDEREVPVGAVLVLNNRVIGEGWNRAIGLHDPTAHAEIMALRQGGLVMQNYRLIDATLYVTFEPCVMCAGAMIHSRIGRVVFGVRNNKHGAAGSLVNVLNYPGMNHRVEITEGILVDECAALLCDFYRMSRQVLNAQKKAQSSISSGGSSGGSSGSETPGASGSVIPKSSGGSSAGSTKDTITKTLKLRIVRPYNSAEVEKIVADEKNSREKIALERNKDKVREACSEHLKVAAYCTTQVERNACLFCKARKLDDRFYQKLRGQFPDAVFWQETGEIFRQLQRQAAEIYNQSLIELYYEIFIKGKGFANASSVEHYLSDVCYTRAAELFKNAAIASGLRNKIKSNFRLKELRNMKSGLPTTKSDNFPIPLVRQKGGQYTGFEISNHNGDFIIKIPFGRWQVKKEIDKYRPWEKFDFAQVRKSPKPISLLLSTQRRKRNRGWSKDEGTEAEIKKVMNGDYQTSYIEVKRGSKIGEKSAWMLNLSIDVPKIDKGVDPSIIGGIDVGVKSPLVCAINNAFSRYSISDNDLFHFNKKMFARRRILLKKNRHKRAGHGAKNKLKPISILTEKSKRFRKKLIERWACEIADFFVKNKVGTVQMENLESMKRKEDSYFNIRLRGFWPYAEMQNKIELKLKQYGIKIRKVAPNNTSKTCSKCGHLNDYFNFEYRKKNKFPHFKCEKCNFKEDADYNAALNISNPKLKSTREVP

SEQ ID NO: 2424 - protein, 726 aa, synthetic construct
SEVEFSHEYWMRHALSLAKRARDEREVPVGAVLVLNNRIIGEGWNRAIGLHDPTAHAEIMALRQGGLVMQNYRLTDATLYVTFEPCVMCAGAMVHGRIGRVVFGVRNSKRGAAGSLMNVLNYPGVNHCVEITEGILVDECAALLCDFYRMPRQVLNAQKKAQSSISSGGSSGGCSGSEMPGASESVTPKSSGGSSAGSTKNTITKTLKLRIVRPYNSAEVEKIVADEKNNREKIALEKNKDKVKEACSRHLKVAAYCTTQVERNACLFCKARKLDDKFYRKLKGQFPDAVFWQEIGEIFRQLQKQAAEIYNQSLIELYYEIFIKGKGFANASSVEHYLSDVCYTRAAELFKNAAIASGLRGKVKSNFRLKELKNMKSGLPTTKSDNFPIPLVKQKGGQYTGFEISSHNDDFIIKIPFGRWQVKKEIDKYRPWEKFDFEQVRKSPKPISLLLSTQRRKRNKGWSKDEGTEAEIRKVMNGDYQTSYIEVKRGSKIGEKSAWMLNLSIDVPKIDKGVDPSIIGGIDVGVKSPLVCAINNAFSRYSIGDNDLFHYNKKMFARRRILLKKNRHKRAGHGAKNKLKPTSILTEKSKRFRKKLIERWACEIADFFIKNKVGTVQMENLEGMKRKEDSYFNIRLRGFWPYAEMQNKIEFKLKQYGIEIRKVAPNNTSKTCSKCGHLNNYFSFEYRKKNKFPHFKCEKCNFKEDADYNAALNISNPKLKSTKEEP

SEQ ID NO: 2425 - protein, 726 aa, synthetic construct
SEVEFSHEYWMRHALTLAKRARDEREVPVGAVLVLNNRVIGEGWNRAIGLHDPTAHAEIMALRQGGLVMQNYRLTDATLYVTFEPCVMCAGAMIHSRIGRVVFGVRNSKRGAAGSLMNVLNYPGMNHCVEITEGILVDECAALLCDFYRMPRQVLNAQKKAQSSISSGGSSGGSSCSETSGASESVTPKSSGGSSAGTTKNTITKTLKLRIVRPYNSAEVEKIVADEKNSREKIALEKNKDKVKEACSKHLEVAAYCTTQVERNACLFCKARKLDDKFYQKLRGQFPDAVFWQELGVIFRQLQKQAAEIYNQSLIELYYEIFIKGKGFTNASSVEHYLSDVCYTRAAELFKNAAIASGLRGKVKSNFRLKELKNMKSGLPTTKSDNFPIPLVKQKGGQYTGFEISSHNDDFIIKIPFGRWQVKKEVDKYRPWEKFDFEQVRKSPKPISLLLSTQRRKRNKGWSKDEGTEAEIRKVMNGDYQTSYIEVKRGSKIGEKSAWMLSLSIDVPKIDKGVDPSIIGGIDVGVKSPLVCAINNAFSRYSISDNDLFRFNKKVFARRRILLKKNRHKRAGHGTKNKLKPIAILAEKSGRFRKKLIERWACEIADFFIKNKVGTVQMENLESMKRKEDSYFNIRLRGFWPYAEMQNRIEFKLKQYGIEIRKVAPNNTSKTCSKCGHLNNYFNFEYRKKNKFPHFKCEKCNFKENADYNAALNISNPKLKSTKEEP

SEQ ID NO: 2426 - protein, 725 aa, synthetic construct
SEVEFSHEYWMRHALTLAKRARDEREVPVGAILVLNNRVIGEGWNRAIGLHDPTAHAEIMALRQGGLVMQNYRLIDATLYVTFEPCVMCAGAMIHSRIGRVVFGVRNNKHGAAGSLVNVLNYPGMNHRVEITEGILADECAALLCDFYRMPRQVLSARKKAQSSVSSGGSSGGSSGSETPGASGSVTPKSSVGSSAGSTKNTITKTLKLRIVRPYNSAEVEKIVADEKNNREKIALEKNRDKVKEACSKHLKVAAYCTTQVERNACLFCKARKLDDKFYQKLRGQFPDAVFWQELGEILRQLQKQAAEIYNQSLIELYYEIFIKGRGFANASSVEHYLSDVCYTRAAELFKNAAIASGLRGKVKSNFRLKELKNMKSGLPTTKSDNFPIPLVKQKGGQYTGFEISSHNDDFIIKIPFGRWQVKKEIDKYRPWEKYDFEQVRKSPKPISLLLSTQRRKRNKGWSKDEGTEAEIRKVMNGDYQTSYIEVKRGSKTGEKSAWMLNLSIDVPRIDKGVDPSIIGGIDVGVKSPLVCAINNAFSRYSISDNDLFRFNKKMFARRRILLRKNRHKRAGHGAKNKLKPISILTGKSERFRKKLIERWACEIADFFIKNRVGTVQMENLESMKRKEDSYFNIRLRGFWPYAEMNKIEFKLKQYGIEIRKVAPNNTSKTCSKCGHLNNYFNFEYRKKNKFPHFKCEKCNFKENADYNAALNISNPKLKSTKEEP

SEQ ID NO: 2427 - protein, 726 aa, synthetic construct
SEVEFSHEYWMRHALTLAKRARDEREVPVGAVLVLNNRVIGEGWNRAIGLHDPTAHAEIMALHQGGLVMQNYRLIDATLYVTFEPCVMCAGAMIHSRIGRVVFGARNSKRGAAGSLMNVLSYPGMNHRVEITEGILADECAALLCDFYRMPRRVFNAQKKAQSSINSGGSSGGGSSSDTPSTSESTTPESSGGSSGGPAKNTITKTLKLRIVRPYNSAEVEKIVADEKNNREKTALEKNKDKVKEACSKHLKVAAYCTTQVERNACLFCKARKLDDKFYQRLRGQFPDAVFWQEVGEILRQLQKQAAEIYNQSLIELYYEIFIKGKGFANASSVEHYLSDVCYTRAAELFKNAAIASGLRGKVKSNFRLKELKNMKSGLPTTKSDNFPIPLVKQKGGQYTGFEISNRNSDFIIKIPFGRWQVKKEINKYRPWEKFDFEQVRKSPKPISLLLSTQRRKRNKGWSKDEGTEAEIRKVMNGDYQTSYIEVKRGSRIGEKSAWMLSLSIDVPKIDRGVDPSIIGGIDVGVKSPLVCAINNALSRYSISDNDLFHFNKKMFARRRILLRKNRHKRAGHGARNKLKPITVLTEKSERFRKKLIERWACEIANFFIKNKVGTVQMENLESMKRREDSYFNIRLRGFWPYAEMQSKIEFKLKQYGIKIRKVAPNNTSKTCSKCGHLNNYFNFEFRKKNKFPHFKCEKCNFKEDADYNAALNISNPKLKSTKEEP

SEQ ID NO: 2428 - protein, 726 aa, synthetic construct
SEVEFSHEYWMRHALTLAKRARDEREVPVGAILVLNNRVIGEGWNRAIGLHDPTAHAEIMALRQGGLVMQNYRLVDATLYVTFEPCVMCAGAMIHSRIGRVVFGVRNNKHGAAGSLVNVLNYPGMNHRVEITEGILANECAALLCDFYRMPRQVFNARKKAHSSISSGGSSGGSGGGETPGASESVTPKNSGGSSAGSTKNTITKTLKLRIVRPYNSAEVEKIVADEKNNREKIALEKNKDKVREACSKHLKVASYCTTQVERNACPFCKARKLDNKFYQRLRGQFPDAVFWQEISEIFRQLQKQAAEIYNQSLIELYYEIFIKGKGITNACRVEHYLSDVCYTRAAELFRNAAIASGLRSKVKSNFRLKELKNMRSGLPTTKSDNFPIPLVKQKGGQYTGFEISNHNSDFVIKIPFGRWQVKKEIDKFRPWEKFDFEQVRKSPKPISLLLSTQRRKRNKGWGKDEGTEAEIKKVMNGDYQTSYIEVKRGSKIGEKSAWVLNLSIDVPKIDKGVDPSIIGGIDVGVKSPLVCAINNSSSRYSICDNDLFRFNKKMFARRRILLKKNRHKRAGHGAKNKLKPITILTKKSERFRKKLIERWVCEVADFFIKNKVGTVQMENLESMKRKEDSYFNIRLRGFWPYAEMQNRIELKLKQYGIEIRRVAPNNTSRTCSKCGHLNNYFNFEYRKKSKFPHFKCEKCNFREDADYNAALNISNPKLRSTKEEP

SEQ ID NO: 2429 - protein, 726 aa, synthetic construct
SEVEFSHEYWMRHALTLAKRARDEREVPVGAVLVLDNRVIGEGWNRTTGLHDPTAHAEIMALRQGGLVMRNYRLTDATLYVTFEPCVMCAGAMIHSRIGRVVFGVRNSKRGAAGSLMNVLNYPGMNHRVEITEGILVDECAALLCDFYRMPRQVFSAQKKAQSTINSGGSSGGSSGSETPGTSESATPESSGGGSSGSAKNTITKTLQLRIVRPYNSAEVEKIVADEKNNREKIALEKNKDKVREACSKHLKVASYCTTQVERNACLFCKARKLDDKFYQRLRGQFPDAVFWQELGGIFRQLQKQAAEIYNQSLIELYYEIFIKGKGITNASRVEHYLSDVCYTRAAELFKNAAIASGLRSKVRSNFRLKELKNMKSGLPTTKSDNFPIPLVKQKGGQYTGFEISSHNSDFIIKIPFGRWQVKEEIDKYRPWEKFDFEQVRKSPKPISLLLSTQRRQKNKGWSKDEGTEAEIRRVMNGDYQTSYIEVKRGSKIGEKSTWMLNLSIDVPKIDKGVDPSIVGGIDVGVKSPLVCAINNSFSRYSICDNDLFRFNKKMFARRRILLRKNRHKRAGHGAKNKLKPITILTKKSERFRKKLIERWVCEVADFFIKNKVGTVQMENLESMKRKEDSYFNIRLRGFWPYAEMQNRIELKLKQYGIEIRKVAPNNTSRTCSKCGHLNNYFNFEYRKKNKFPHFKCEKCNFKENADYNAALNISNPKLKSTKEKP

SEQ ID NO: 2430 - protein, 726 aa, synthetic construct
SEVEFSHEYWMRHALTLARRARDEREVPVGAILVLNNRVIGEGWNRAIGLHDPTAHAEIMALRQGGLVMQNYRLIDATLYVTFEPCAMCAGAMIHGRIGRVVFGVRNNKHGAAGSLMNVLNYPGMDHRVEITEGILADECAALLCDFYRMPRQVFNARKKAQSGINPGGSPGGSSGSETPGTSESATPEGSGGSSGGSAKNTITKTLKLRIVRPYNSAEVERIVADEKNNREKIALEKNKDKVKEACSEHLKVAAYCSTQVERNACLFCKARKLDDKFYQKLRGQFPDAVFWQEIGEIFRQLQKQAAEIYNQSLIELYYEIFIKGKGIANASSVGHYLSDVCYTRAAELFKNAAIASGLRGKIKSNFRLKELKNMKSGLPTTKSDNFPIPLVKQKGGQYTGFEISNHNSDFIIKIPFGRWQVKKEIDKHRPWEKFDFEQVRKSPKPISLLLSTQRRKRNKGWSKDEGTEAEIKKVMNGDYQISYIEVKRGSKIGEKSAWMLNLSIDVPKIDKGVDPSIIGGIDVGVKSPLVCAINNAFSRYSISDNDLFHFNKKMFARRRILLKKNGHKRAGHGVKNKLKPITILTEKSGRFRKKLIERWACEIADFFIKNKVGTVQMENLESMKRREDSYFNIRLRGFWPYAEMQNKIEFKLKQYGIEIRKVAPNNTSKTCSKCGHLNNYFNFEYRRKNKFPHFKCEKCNFKENADYNAALNISNPKLKSTKEEP

SEQ ID NO: 2431 - protein, 726 aa, synthetic construct
SEVEFSHEYWMRHALTLAKRARDEREVPVGAVLVLNNRVIGGGWNRAIGLHDPTAHAEIMALRQGGLVMQNCRLVDATLYVTFEPCVMCAGAMIHSRIGRVVFGVRNSKRGAAGSLMNVLNYPGMNHRVEITEGILAGECAALLCDFYRMPRQVFNAQKKAQSTISSGGSSGGSSGSETPGTSGSATPEGSGGSSGGSAKNTITKTLKLRIVRPYNSAEVEKIVADEKNNREKIALEKNKDKVKEACSKHLKVAAYCTTQVERNACLFCKARKLDDKFYQKLRGQFPDAVFWQEIGEIFRQLQKQAAEIYNQSLIELYYEIFIKGKGFANASSVEHYLSDVCYTRAAELFKNAAIASGLRGKVKSNFRLKELKNMRSGLPTTKSDNFPIPLVKQKGGQYTGFEISSHNDDFIIKIPFGRWQVKKEIDKYRPWEKFDFEQVRRSPKPISLLLSTQRRKKNKGWSKDEGTEAEIRRVMNGDYQTSYIEVKRGSKIGEKSAWMLNLSIDVPKIDKGVDPSIIGGIDVGVKSPLVCAINNAFSRYSISDNDLFHFNKKMFARRRILLKKNRRRRAGHGAKNKLKPITILTEKSVRFRKKLIERWACEIAHFFIKNKVGTVQMENLEGMKRREDSYFNIRLRGFWPYAEMQNRIEFKLKQYGIEIRKVAPNNTSKTCSKCGHLNNYFNFEYRKKNKFPHFKCEKCNFKENADYNAALNISNPKLKSTKEEP

SEQ ID NO: 2432 - protein, 726 aa, synthetic construct; identical to SEQ ID NO: 684

SEQ ID NO: 2433 - protein, 726 aa, synthetic construct
SEDEFSHEYWMRHALTLAKRARDGREVPVGAVLVLNNRVIGEGWNRAIGLHDPTAHAEIMALRQGGLVMQNYRLIDATLYVTFEPCVMCAGAMVHSRIGRVVFGVRNSKRGAAGSLMNVLDYPGMGHRVEITEGILADECAALLCDFYCMPRQVFNAQKRAQSSINSGGSSGGSCGSDTPGTSESATPKSSGGSSGGSAKNTITKTLKLRIVRPYNSAEVEKIVADEKNNREKIALEKNKDKVKEACSKHLKVAAYCTTQVERNACLFCKARKLDDKFYQELRGQFPDAVFWQEIGEIFRQLQKQAAEIYNQSLIELYYEIFIKGRGFANASSVEHYLSDVCYTRAAELFKNAAIASGLRNKIKSNFRLKELRNMKSGLPTTKSDNFPIPLVRQKGGQYTGFEISNHNGDFIIKIPFGRWQVKKEIDKYRPWEKFDFEQVRKSPKPISLLLSTQRRKRNKGWSKDEGTEAEIRKVMNGDYQTSYIEVKRGSKTGEKSAWMLNLSIDVPKIDKGVDPSIIGGIDVGVKSPLVCAINNTFSRYSISDNDLFRFNKKMFARRRILLKKNRHKRAGHGAKNKLKPISILTGKSERFRKRLIERWACEIADFFIKNKVGTVQMENLESMKRKEDSYFNIRLRGFWPYAEMQNKIEFKLKQYGIGIRKVAPNNTSKTCSKCGHLNNYFNFEYRKKNKFPHFKCERCNFKENADYNAALNISNPKLKSTKEKP

SEQ ID NO: 2434 - protein, 726 aa, synthetic construct
SEVEFSHEYWMRHALSLAKRARDEREVPVGAVLVLNNRIIGEGWNRAIGLHDPTAHAEIMALRQGGLVMQNYRLTDATLYVTFEPCVMCAGAMVHGRIGRVVFGVRNSKRGAAGSLMNVLNYPGMNHCVEITEGILVDECAALLCDFYRMPRQVLNAQKKAQSSISSGGSSGGSSGSETPGASESVTPKSSGGSSGGSAKNTITKTLKLRIVRPYNSAEVEKIVADEKNNREKIALEKNKDKVKEACSKHLKVAAYCTTLVERNACLFCKARRLDDKFYQKLRGQFPDAVFWQEIGEIFRQLQKQAAEIYNQSLVELYYEIFIKGKGIANASSVEHYLSDVCYTRAAELFKNAAIASGLRNKIKSNFRLKELRNMKSGLPTTKSDNFPIPLVRQKGGQYTGFEISSHNSDFIIKIPFGRWQEKEEIDKYRPWEKFDFEQVRRSPKPISLLLSTQRRKKNKGWSKDEGTEAEIRRVMNGDYQTSYIEVKRGSKIGEKSAWMLNLSIDVPKIDKGVDPSIIGGIDVGVKSPLICAINNAFSRYGISDNDLFRFNKKMFARRRILLGKNRHQRAGHGAKNKLKPITILTEKSGRFRKKLIERWACEIADFFVKNKVGTVQMENLESMKRKEDSYFNIRLRGFWPYAEMQNKIEFKLKQYGIKVRKVAPNNTSKTCSKCGHLNNYFSFEYRKRNKFPHFKCEKCNFKENADYNAALNISNPKLKSTKEEP

SEQ ID NO: 2435 - protein, 726 aa, synthetic construct; identical to SEQ ID NO: 684

SEQ ID NO: 2436 - protein, 726 aa, synthetic construct
SEVEFSHEYWMRHALTLAKRARDEREVPVGAILVLNNRVIGEGWNRAIGLHDPTAHAEIMALRQGGLVMQNHRLIDATLYVTFEPCVMCAGAMIHSRIGRVVFGVRNNKHGAAGSLVNVLNYPGMNHRVEITEGILADECAALLCDFYRMPRQVFNAQKKAQSSISSGGSSGGSSGSETPGASGSVIPKSSGGSSDGSAKNTITKTLKLRIVRPYNSAEVEKIVADEKNNREKIALEKNKDKVKEACSKHLKVAAYCTTQVERNACLFCKARKLDDKFYQKLRGQFPDAVFWQELGEIFRQLQKQAAVIYNQSLIELYYEIFIKGKGIANASRVEHYLSDVCYTRAAELFKNAAVASGLRGKVKSNFRLKELKNMKSGLPTTKSDNFPIPLVKQKGGQYTGFEISSHNDDFIIKIPFGRWQVKKEINKHRPWEKFDFEQVRKSPKPISLLLSTQRRKRNKGWSKDEGTEAEIRKVMNGDYQTSYIEVKRGSKIGEKSAWMLNLSIDVPKIDKGVDPSIIGGIDVGVKSPLVCAINNAFSRYSISDNDLYRFNKKMFARRRILLKKNRHKRAGHGAKNKLKPISILTERSRRFRKKLIERWACEIADFFIRNKVGTVQMENLESMKRKEDSYFNIRLRGFWPYAEMQNKIEFKLKQYGIEIRRVAPNNTSKTCSKCGHLNNYFNFEYRKKNKFPYFKCEKCNFKENADYNAALNISNPKLKSTKEEP

SEQ ID NO: 2437 - protein, 726 aa, synthetic construct; identical to SEQ ID NO: 684

SEQ ID NO: 2438 - protein, 726 aa, synthetic construct
SEAEFSHEYWMRHALTLAKRARDEREVPVGAVLVLNNRVIGEGWNRAIGLHDPTAHAEIMALRQGGLVMQNYRLIDATLYVTFEPCVMCAGAMIHSRIGRVVFGVRNSKRGAAGSLMNVLNYPGMNHRVEITEGVLADECAALLCDFYRMPRQVLNAQKKAQSSINSGGSSGGGSGGETPGTSESATQESSGGSSAGSTKDTITKTLKLRIVRPYNSAEVEKVVADEKNNREKIAMEKNKDKVKEACSKHLKVASYCTTQVERNACLFCKARKLDDKFYQKLRGQFPDAVFWQELGGIFRQLQKQAAEIYNQSLIELYYEIFIKGKGITNASRVEHYLSNVCYTRAAELFKNAAIASGLRSKVRSNFRLKELKNMKSGLPTTKSDNFPIPLVKQKGGQYTGFEISSHNSDFIIKIPFGRWQEKEEIDKYRPWEKFDFEQVRRSPKPISLLLSTQRRKKNKGWSKDDGTEAEIRRVMNGDYQTSYIEVKRGSKIGERSAWMLNLSIDVPKIDKGVDPSIIGGIDVGVKSPLVCAINNAFSRYSISDNDLFHFNKKMFARRRILLKKNRRRRAGHGAKNKLKPITILTEKSVRFRKKLIERWACEIADFFIKNKVGTVQMENLESMKRKEDSYFNIRLRGFWPYAEMQNKIEFKLKQYGIEIRRVAPNNTSRTCSKCGHLNNYFNFEYRRKYKFPHFKCEKCNFKEDADYNAALNISNPKLKSTKEEP

SEQ ID NO: 2439 - protein, 726 aa, synthetic construct
SEVEFSHEYWMRHALTLAKRARDEREVPVGAVLVLDNRVIGVGWNRAIGLHDPTAHAEIMALRQGGLVMQNYRLTDATLYVTFEPCVMCAGAMVHSRIGRVVFGVRNSKRGAAGSLMNVLNYPGMSHCVEITEGILVDECAALLCDFYRMPRQVLNAQKKAQSSISSGGSSGGSSCSETPGASESVTPKSSGGSSAGSTKNTITKTLKLRIVRPYNSAEVEKIVADEKNSREKIALEKNKDKVKEACSEHLKVAAYCTTQVERNACLFCKARKLDDRFYQKLRGQFPDAVFWQEIGEIFRQLQKQAAEIYNQGLIELYYEIFIEGKGIANASRVEHYLSNVCYTRAAELFKNAAIASGLRNKIKSNFRLKELRNMKSGLPTTKSDNFPIPLVRQKGGQYTGFEISNHDGDFIIKIPFGRWRVKKEINKHRPWEKFDFEQVRKSPKPISLLLSTQRRKRNKGWSKDEGTEAEIRKVMNGDYQTSYIEVKRGSKIGEKSAWMLNLSIDVPKIDKGVDPGIIGGIDVGVKSPLVCAINSASSRYSISDNDLFHFNKKMFARRRVLLKKNGHKRAGHGAKNKLKPITIMTEKSKRFRKKLIERWACEVADFFIKNKVGTVQMENLGSMKRKEDSYFNIRLRGFWPYAEMQNKIEFKLKQYGIEIRKVAPDNTSKTCSKCGHLNNYFNFEYRKKNKFPHFKCEKCNFKEDADYNAALNISNPKLKSTKEEP

SEQ ID NO: 2440 - protein, 726 aa, synthetic construct
SEVEFSHEYWMRHALSLAKRARDEREVPVGAVLVLNNRIIGEGWNRAIGLHDPTAHAEIMALRQGGLVMQNYRLTDATLYVTFEPCVMCAGAMVHSRIGRVVFGVRNSKRGAAGSLMNVLNYPGVNHRVEITEGILVDECAALLCDFYRMPRQVLNAQKKAQSSISPGGSSGGCSGSEMPGASESVTPESSGGSPGGSAKNTITKTLKLRIVRPYNSAEVEKIVADEKNNREKIALEKNKDKVKEACSKHLKVAAYCTTQVERNACLFCKARKLDDKFYQKLRGQFPDAVFWQEIGEIFRQLQKQAAEIYNQSLIELYYEIFIKGKGFANASSVEHYLSDVCYTRAAELFKNAAIASGLRGKVKSNFRLKELKNMKSGLPTTKSDNFPIPLVKQKGGQYTGFEISSHNDDFIIKIPFGRWQVKEEIDKYRPWEKFDFEQVRKNPKPISLLLSTQRRKGNKGWSKDEGTEAEIRKVMNGDYQTSYIEVKRGSKIGEKSAWMLNLSIDVPKIDKGVDPSIIGGIDVGVKSPLVCAISNAFSRYSISDNDLFHFNKKMFARRRILLKKSKHKRAGHGAKNKLKPITILTEKSRRFRKKLIERWACEIADFFIKNKVGTVQMENLESMKRKEDSYFNIRLRGFWPYAEMQNKIEFKLKQYGIEIRKVAPNNTSKTCSKCGHLNNYFNFEYRKKNKFPHFKCEKCNFKENADYNAALNISNPKLKSTKEEP

SEQ ID NO: 2441 - protein, 726 aa, synthetic construct
SEVEFSHEHWMRHALTLAKRARDEREVPVGAVLVLNNRVIGEGWNRTTGLHDPTAHAEIMALRQGGLVMQNYRLIDATLYVTFEPCVMCAGAMIHSRIGRVVFGVRNNKHGAAGSLVNVLNYPGMNHRVEITEGILADECAALLCDFYRMPRQVFNARKKAQSSINPGGSSGGSSGSETPSTSESTTPESSGGSSGGPAKNTTTKTLKLRIVRPYNSAEVEKIVADEKNNREKTALEKNKDKVKEACSKHLKVAAYCTTLVERNACLFCKARKLDDKFYQKLRGQFPDAVFWQEVGEIFRQLQKQAAEIYNQSLIELYYEIFIKGKGFANASSVEHYLSDVCYTRAAELFKNAAIASGLRNKVKSNFRLKELRNMKSGLPTTKSDNFPIPLVRQKGGQYTGFEISNHDGDFIIKIPFGRWQVKKEINKHRPWEKFDFEQVRKSPKPISLLLSTQRRKRNKGWSKDEGTEAEIRKVMKGDYQTSYIEVKRGSKIGEKSAWMLNLSIDVPKIDKGVDPGIIGGIDVGVKSPLVCAINNVLSRYSISDNDLFHFNKKMFARRRILLKKNGHKRAGHGAKNKLKPITIMTEKSKRFRKKLIERWACEIADFFIKNKVGTVQMENLESMKRKEDSYFNIRLRGFWPYAEMQNKIEFKLKQYGIEIRKVAPNNTSKTCSKCGHLNNYFSFEYRKKNKFPHFKCEKCNFKENADYNAALNISNPKLKSTKEEP

SEQ ID NO: 2442 - protein, 726 aa, synthetic construct
SEAEFSHEYWMRHALTLAKRARDEREVPVGAVLVLNNRVIGEGWNRAIGLHDPTAHAEIMALRQGGLVMQNYRLIDATLYVTFEPCVMCAGAMVHSRIGRVVFGVRNSKRGAAGSLMNVLDYPGMGHRVEITEGILADECAALLCDFYCMPRQVFNAQKRAQSSINSGGSSGGSSGSETPGASGSVTPKSSGGSSAGSTKDTITKTLKLRIVRPYNSAEVEKIVADEKNSREKIALEKNKGKVKEACSEHLKVAAYCTTQVERNACLFCKARKLDDKFYQKLRGQFPDAVFWQEIGEIFRQLQKQAAEIYNQSLIELYYEIFIKGKGITNASRVEHYLSDVCYSRAAELFKNAAIASGLRSKVRSNFRLKELKNMKSGLPTTKSDNFPIPLVKQKGGQYTGFEISSHNSDFIIKIPFGRWQVKEEIDKYRPWEKFDFEQVRKSPKPISLLLSTQRRKKNKGWSKDEGTEAEIRRVMNGDYQTSYIEVKRGSKIGEKSAWMLNLSIDVPKIDKGVDPSIIGGIDVGVKSPLVCAINNSSSRYSISDNDLFHFNKKMFARRRILLKKNRHRRAGHGARNKLKPITVLTEKSKRFRKKLIERWACEIANFFIKNKVGTVQMENLESMKRKEDSYFNIRLRGLWPYAEMQNKIEFKLKQYGIEVRKVAPNNTSKTCSKCGHLNDYFNFEYRRKNKFPHFKCEKCNFKENADYNAALNISNPKLKSTKEEP

SEQ ID NO: 2443 - protein, 726 aa, synthetic construct
SEDEFSHEYWMRHALTLAKRARDGREVPVGAVLVLNNRVIGEGWNRAIGLHDPTAHAEIMALRQGGLVMQNYRLIDATLYVTFEPCVMCAGAMVHSRIGRVVFGVRNSKRGAAGSLMNVLDYPGMGHRVEITEGILADECAALLCDFYCMPRQVFNAQKRAQSSINSGGSSGGSSGSDTPGTSESATPESSGGGSSGSAKNTITKTLQLRIVRPYNSAEVEKIVADEKNNREKIALEKNKDKVREACSKHLKVASYCTTQVERNACPFCKARKLDDKFYQKLRGQFPDAVFWQEIGEIFRQLQKQAAEIYNQSLIELYYEIFIKGKGFANASSVEHYLSDVCYTRAAELFKNAAIASGLRGKVKSNFRLKELKNMKSSLPTTKSDNFPIPLVKQKGGQYTGFEISSRNDDFIIKIPFGRWQAKKEIDKYRPWEKFDFEQVRKSPKPISLLLSTQRRKRNRGWSKDEGTEAEIRKVMNGDYQTSYIEVKRGSKIGEKSAWMLNLSIDVPKIDKGVDPSIIGGIDVGVKSPLVCAINNAFSRYSISDNDLFRFNKKMFARRRILLKKTRHKRAGHGAKNKLKPISILTEKSERFRKKLIERWACEIADFFIKNKVGTVQMENLESMKRKEDSYFNIRLRGFWPYAEMQNKIEFKLKQYGIEIRKVAPNNTSKTCSKCGHLNNYFNFEYRKMNKFPHFKCERCNFKENADYNAALNISNPKLKSTKEEP

SEQ ID NO: 2444 - protein, 726 aa, synthetic construct
SEVEFSHEYWMRHALTLAKRARDEREVPVGAVLVLNNRVIGEGWNRAIGLHDPTAHAEIMALRQGGLAMQNYRLVDATLYVTFEPCVLCAGAMVHSRIGRVVFGVRNSKRGAAGSLMNVLNHPGMNHRVEITGGILADECAALLCDFYRMPRQVFNAQKKARSNINSGGSSGGSSDSETPGASGSVTPKSSGGSSAGSTKDAITKTLKLRIVRPYNSAEVEKIVADEKNNREKIAMEKNKDKVKEACSKHLKVASYCTTQVERNACLFCKAGKLDDKFYQKLRGQFPDAVFWQELGGIFRQLQKQAAEIYNQSLIELYYEIFIKGKGITNASRVEHYLSDVCYTRAAELFKNAAIASGLRSKVRSNFRLKELKNMKSGLPTTKSDNFPIPLVKQKGGQYTGFEISSHNSDFIIKIPFGRWQEKEEIDKYRPWEKFDFEQVRKSPKPISLLLSTQRRKKNKGWSKDEGTEAEIRKVMNGDYQTSYIEVKRGSKIGEKSAWMLNLSIDVPRIDKGVDPSIIGGIDVGVKSPLVCAINNAFGRYSISDNDLFHFNKKMFARRRILLKKNRHKRAGHGAKNKLKPITILTEKGKRFRKKLIERWACEIADFFIKNKVGTVQMENLESMKRKEDSYFNIRLRGFWPYAEMQDKIEFKLKQYGIEIRKVAPNNTSKTCSRCGHLNDYFNFEYRRKNKFPHFKCEKCNFKENADYNAALNISNPKLKSTKEEP

SEQ ID NO: 2445 - protein, 726 aa, synthetic construct
NEVEFSHEYWMRHALTLAKRARDEREVPVGAVLVLNNRAIGEGWNRTAGLHDPTAHAEIMALRQGGLVMQNHRLVDATLYVTFEPCVMCAGAMIHSRIGRVVFGVRNSKRGAAGSLMNVLNHPGMNHRVEITEGILVDECAALLCDFYRMPCQVLNAQKKAQSSISSGGSSGGSSGGDTLGASESVTPKSSVGSSASSTKNTITKTLKLRIVRPYNSAEVEKIVADEKNNREKIALEKNEDKVKEACSEHLKVAAYRTTQVERSACLFCKARKLDDKFYQKLRGQFPDAVFWQEIGEIFRQLQKQAAEIYNQSLIELYYEIFIKGKGFANASSVEHYLSDVCYTRAAELFKNAAIASGLRGKVKSNFRLKELKNMKSGLPTTKSDNFPIPLVKQKGGQYTGFEISSHNDDFIIKIPFGRWQAKKEIDKYRPWEKFDFEQVRKSPKPISLLLSTQRRKRNKGWGKDEGTEAEIRKVMNGDYQTSYIEVKRGSKIGEKSAWMLNLSIDVPKIDKGVDPSIIGGIDVGVKSPLVCAINNALSRYSISDNDLFHFNKKMFARRRILLKKNRHKRAGHGAKNKLKPITILTEKSKRFRKKLIERWACEIADFFIKNKVGTVQMENLESMKRKEDSYFNIRLRGFWPYAEMQNKIEFKLKQYGIEIRKVAPNNTSKTCSKCGHLNDYFNFEYRRKNKFPHFKCEKCNFKEDADYNAAQNISNPKLKSTKEEP

SEQ ID NO: 2446 - protein, 726 aa, synthetic construct
SEVEFSHEYWMRHALTLAKRARDVREVPVGAVLVLNNRVIGEGWNRAIGLHDPTAHAEIMALRQGGLVMQNYRLVNATLYVTFEPCVMCAGAMIHSRIGRVVFGVRNSKRGAAGSLMNVLNYPGMNHRVEITEGILTDECAALLCDFYRMPHQVLSAQKKAQSSINSGGSSGGSSGSETPGTSGSATPEGSGGSSGGFAKNTITKTLKLRIVRPYNSAEVEKIVADEKNNREKIALEKNKDKVKEACSKHLKVAAYCTTQVERNACLFCKARKLDDKFYQRLRGQFPDAVFWQELGEIFRQLQKQAAEIYNQSLIELYYEIFIKGKGFANASSVEHYLSDVCYTRAAELFKNAAIASGLRGKVKSNFRLKELKNMKSGLPTTKSDNFPIPLVKQKGGQYTGFEISSHNDDFIIKIPFGRWQVRKEIDKYRPWEKFNFEQVRKSPKPISLLLSTQRRQKNKGWSKDEGTEAEIRRVMNGDYQTSYIEVKRGSKIGEKSTWMLNLSIDVPKIDKGVDPSIVGGIDVGVKSPLVCAINNSFSRYSICDNDLFRFNKKMFARRRILLKKNRHKRAGHGAKNKLKPITILTKKSERFRKKLIERWVCEVADFFIKNKVGTVQMENLESMKRKEDSYFNIRLRGFWPYAEMQNRIELKLKQYGIEIRRVAPNNTSRTCSKCGHLNNYFNFEYRKKNKFPHFKCEKCNFREDADYNAALNISNPKLKSTKGEP

SEQ ID NO: 2447 - protein, 726 aa, synthetic construct; identical to SEQ ID NO: 684

SEQ ID NO: 2448 - protein, 726 aa, synthetic construct
SEVEFSHEYWMRHALTLAKRARDEREVPVGAILVLNNRVIGEGWNRAIGLHDPTAHAEIMALRQGGLVMQNYRLIDATLYVTFEPCVMCAGAMIHSRIGRVVFGVRNNKHGAAGSLVNVLNYPGMNHRVEITEGILADECAALLCDFYRMPRQVFNARKKAQSSINPGGSSGGSGGSETPGTSESPTPESSGGSSGGSAKNTITKTLKLRIVRPYNSAEVEKIVAEEKDNREKIALEKNKDKVREACSKHLKVASYCTTQVERNACPFCKARKLDDKFYQKLRGQFPDAVFWQELGEILRQLQKQAAEIYNQSLIELYYEIFIKGRGFANASSVEHYLSDVCYTRAAELFKNAAIASGLRGKVKSNFRLKELKNMKSGLPTTKSDNFPIPLVKQKGGQYTGFEISSRNDDFIIKIPFGRWQVKKEIDKYRPWEKFDFEQVRKSPKPISLLLSTQRRKRNKGWGKDDGTEAEIRKVMNGDYQTSYIEVKRGSKTGEKSAWMLNLSIDVPKIDKGVDPSIIGGIDVGVKSPLVCAINNAFSRYSISDNDLFRFNKKMFARRRVLLKKNRHKRAGHGAKNKLKPISILTGKSKRFRKKLIERWACEIADFFIKNKVGTVQMENLESMKRREDSYFNIRLRGFWPYAEMQNKIEFKLKQYGIEIRKVAPNNTSKTCSKCGHLNNYFSFEYRRKNRFPHFKCEKCNFKENADYNAALNISNPKLKSTKEEP

SEQ ID NO: 2449 - protein, 726 aa, synthetic construct
SEVEFSHEYWMRRALTLAKRARDEREVPVGAVLVLNNRVIGVGWNRAVGLHDPTAHAEIMALRQGGLVMQNYRLIEATLYVTFEPCIMCAGAMIHSRIGRVVFGVRNSKRGAAGSLMNVLNYPGMNHRVEITEGILADECAALLCDYYRMPHQVFNARKKAQSSINSGGSSDGGSGSVTPGTSESATPESSGGSSGGSAKNTITKTLKLRIVRPYNSAEVEKIVADEKNNREKVALEKNKDKVKEACSKHLKVAAYCTTQVERNACLFCKARRLDDKFYQKLRGQFPDAVFWQEIGEIFRQLQKQAAEIYNQSLIELYYEIFIKGKGVANANNVEHYLSDVCYTRAAELFKNAAIASGLRNKIKSNFRLKELRNMKSGLPTTKSDNFPIPLVKQKGGQYTGFEIGNHNSDFIIKIPFGRWQAKKEIDKYRPWEKFDFEQVRKSPKPISLLLSTQRRRRNKGWSKDEGTEAEIRKVMNGDYQTSYIEVKRGSKIGEKGAWMLNLSIDVPRIDKGVDPSIIGGIDVGVKSPLVCAINNALSRYSIGDNDLFHFNKKMFARRRILLKKNRHKRAGHGARNKLKPITVLTEKSERFRKKLIERWACEIAYFFIKNKVGTVQMENLESMKRREDSYFNTRLRGFWPYAEMQNKIEFKLKQYGIEVRKVAPNNTSKTCSKCGHLNNYFNFEYRKKNKFPHFKCEKCNFKEDADYNAALNISNPRLKSTKEEP

SEQ ID NO: 2450 - protein, 726 aa, synthetic construct
SEVEFSHEYWMRHALALAKRARDEREVPVGAVLVLNNRVIGEGWNRAIGLHDPTAHAEIMALRQGGLVMQNYRLVNATLYVTFEPCVMCAGAMIHSRIGRVVFGVRNSKHGAAGSLVNVLNYPGMNHRVEITEGILADECAALLCDFYRMPRQVFNARKKAQSSINSGGSSGGSSGSETPGTSESATPKSSGGSSGGSAKNTITKALKLRIVRPYNSAEVEKIVADEKNNREKIALEKNKDKVKEACSKHLKVASYCTTQVERNACLFCKARKLDDRFYQKLRGQFPDAVFWQETGEIFRQLQRQAAEIYNQSLIELYYEIFIKGKGFANASSVEHYLSDVCYTRAAELFKNAAIASGLRGKVKSNFRLKELKNMKSGLPTTKSDNFPIPLVKQKGGQYTGFEISSHNDDFIIKIPFGRWQEKEEIDKYRPWEKFDFEQVRKSPKPISLLLSTQRRKKNKGWSKDEGTEAEIRRVMNGDYRTSYIEVKRGSKIGEKSAWMLNLSIDVPKIDKGVDPSIIGGIDVGVKSPLVCAINNAFSRYSISDNDLFRFNKKMFARKRILLKKNRHKRAGHGAKNKLKPISILTGKSERFRKKLIERWACEIADFFIKNRVGTVQMENLESMKRKEDSYFNIRLRGFWPYAEMQNKIEFKLKQYGIEIRKVAPNNTSKTCSKCGHLNNYFNFEYRKKNKFPHFKCEKCNFKENADYNAALNISNPKLKSTKEKP

SEQ ID NO: 2451 - protein, 726 aa, synthetic construct; identical to SEQ ID NO: 684

SEQ ID NO: 2452 - protein, 726 aa, synthetic construct
SEVEFSHEYWMRHALTLAKRARDEREVPVGAVLVLNNRAIGEGWNRAIGLHDPTAHAEIMALRQGGLVMQNYRLTDATLYVTFEPCVMCAGAMIHSRIGRVVFGVRNSKRGAAGSLMNVLNYPGMNHCVEITEGILVDECAALLCDFYRMPRQVLNAQKKAQSSISSGGSSGGSSGSETPGASGSVIPKSSGGSSAGSTKDTITKTLKLRIVRPYNSAEVEKVVADEKNNREKIAMEKNKDKVKEACSKHLKVASYCTTQVERNACLFCKARKLDDKFYQKLRGQFPDAVFWQELGGIFRQLQKQAAEIYNQSLIELYYEIFIKGKGITNASRVEHYLSDVCYTRAAELFKNAAIASGLRSKVRSNFRLKELKSMKSGLPTTKSDNFPIPLVKQKGGQYTGFEVSSHNDDFIIKIPFGRWQVKKEIDKYRPWEKFDFEQVRKSPKPISLLLSTQRRKRNKGWSKDVGTEAEIRKVMNGDYQTSYIEVKRGSKIGEKSAWMLSLSIDVPKIDRGVDPSIIGGIDVGVKSPLVCAINNASSRLSISDNDLFRFNKKMFARRRILLKKNGHKRTGHGAKNKLKPITILTEKSARFRKKLIERWACEIADFFIRNKVGAVQMENLESMKRKEDSYFNVRLRGFWPYAEMQNKIEFKLKQYGIEIRKVAPNNTSKTCSKCGHLNSYFNFEYRKKNKFPHFKCEKCNFKENADYNAALNISNPKLRSTKEEP

SEQ ID NO: 2453 - protein, 726 aa, synthetic construct
SEVEFSHEYWMRHALSLAKRARDEREVPVGAVLVLNNRIIGEGWNRAIGLHDPTAHAEIMALRQGGLVMQNYRLTDATLYVTFEPCVLCAGAMVHSRIGRVVFGVRNSKRGAAGSLMNVLNYPGMNHRVEITEGILADECAALLCDFYRMPRQVFNARKKAQSSISSGGSSGGCSGSGTPGTSESATPKSSGGSSSGSAKNTITKTLQLRIVRPYNSAEVEKVVADEKNNREKIALEKNKDKVKEACSKHLKVASYCTTQVERNACPFCKARKLDDKFYQKLRGQFPDAVFWQELGEILRQLQKQAAEIYNQSLIELYYEIFIKGKGFANASSVEHYLSDVCYTRAAELFKNAAIASGLRGKVKSNLRLKELKNMKSGLPTTKSDNFPIPLVKQKGGQYTGFEISSHNDDFIIKIPFGRWQVKKEIDKYRPWEKFDFEQVRKSPKPISLLLSTQRRKKNKGWSKDEGTEAEIRRVMNGDYQTSYIEVKRGSKIGEKSAWMLNLSIDVPKIDKGVDPSIIGGIDVGVKSPLVCAINNSSSRYSICDNDLFHFNKKMFARRRILLRNNRHKRAGHGAKSKLKPITVLTEKGERFRKKLIERWACEIANFFVKNKVGTVQMENLESMRRKEDSYFNVRLRGFWPYAEMQNKIEFKLKQYGIEIRKVAPNNTSKTCSRCGHLNNYFNFEYRRKNKFPLFKCERCNFKENADYNAALNISNPKLKSTKEEP

SEQ ID NO: 2454 - protein, 726 aa, synthetic construct
SEVEFSHEYWMRRALTLAKRARDEREVPVGAVLVLNNRVIGVGWNRAIGLHDPTAHAEIMALRQGGLVTQNYRLIDATLYVTFEPCIMCAGAMIHSRIGRVVFGVRNSKRGAAGSLMNVLDYPGMNHRVEITEGILAGECAALLCDFYRMPRQVFNAQKKAQSNINPGGSSGGSSGSETPGTSESPTPESSGGSSGGSAKNTITKTLKLRIVRPYNSAEVEKIVADEKDNREKIALEKNKDKVKEACSKHLKVAAYCTTQVERNACLFCKARKLDDKFYQKLRGQFPDAVFWQEIGEIFRQLQRQAAEIYNQSLIELYYEIFIKGKGFANASSVEHYLSDVCYTRAAELFKNAAIASGLRGKVKSNFRLKELKNMKSGLPTTKSDNFPIPLVKQKGGQYTGFEIGSHNDDFIIKIPFGRWQVKKEIDKYRPWEKFDFEQVRKSPKPISLLLSTQRRKRNKGWSKDEGTAAEIRKVMNGDYQTSYIEVKRGSKTGEKSAWMLSLSIDVPKIDKGVDPSIIGGIDVGVKSPLVCAINNAFRRYSISDNDLFHFNKKMFARRRILLKKSRHKRAGHGAKNKLKPISILTEKSKRFRKKLIERWACEIADFFIKNKVGTVQMENLESMKRKEDSYFNIRLRGFWPYAEMQNKIEFKLKQYGIEIRKVAPNNTSKTCSKCGHLNNYFNFEYRRKNKFPHFKCEKCNFKEDADYNAALNISNPKLKSTKEKP

SEQ ID NO: 2455 - protein, 726 aa, synthetic construct
SEVEFSHEYWMRHALTLAKRARDEREVPVGAVLVLNNRVIGVGWNRAIGLHDPTAHAEIMALRQGGLVMQNYRLTDATLYVTFEPCVMCAGAMVHSRIGRVVFGVRNSKRGAAGSLMNVLNYPGMSHCVEITEGILVDECAALLCDFYRMPRQVLSAQKKAQSSVSSGGSSGGCSGSEMPGASESVTPKSSGGSSAGSTKNTITKTLKLRIVRPYNSAEVEKIVADEKNSREKIALERNKDRVKEACSEHLKVAAYCTTQVERNACLFCKARKLDDRFYQKLRGQFPDAVFWQETGEIFRQLQRQAAEIYNQSLIELYYEIFIKGKGFANASSVEHYLSDVCYARAAELFKNAAIASGLRGKVKSNFRLRELKNMKSGLPTTKSDNFPIPLVKQKGGQYTGFEISSHNDDFIIKIPFGRWQVKKEIDKYRPWEKFDFEQVRKSPKPISLLLSTQRRKRNKGWSKDEGTEAEIRKVMNGDYQTSYIEVKRGSKTGEKSAWMLNLSIDVPKIDKGVDPSIIGGIDVGVKSPLVCAINNALSRYSISDNDLFHFNKKMFARRRILLRKNRHKRAGHGARNKLRPITVLTEKSERFRKKLIERWACEIANFFIKNKVGTVQMENLESMKRREDSYFNIRLRGFWPYAEMQNKIEFKLKQYGIEIRKVAPNNTSKTCSKCGHLNNYFNFEYRKKNKFPHFKCEECNFKENADYNAALNISNPKLKSTREEP

SEQ ID NO: 2456 - protein, 726 aa, synthetic construct; identical to SEQ ID NO: 684

SEQ ID NO: 2457 - protein, 726 aa, synthetic construct
SEVEFSHEYWMRHALTLAKRARDEREVPVGAILVLNNRVIGEGWNRAIGLHDPTAHAEVMALRQGGLVMQNYRLTDATLYVTFEPCVMCAGAMIHGRIGRVVFGVRNSKRGAAGSLMNVLNYPGMNHCVEITEGILVDECAALLCDFYRMPRQVLNAQKKAQSSISPGGSSGGSSGSETPGASGSVTPKSSGGGSAGSTKDTITKTLKLRIVRPYNSAEVEKIVADEKNSREKIALEKNKDKVKEACSEHLKVAAYCTTQVERNACLFCKARKLDDRFYQKLRGQFPDAVFWQEIGEIFRQLQKQAAEIYNQSLIELYYEIFIKGKGFANASSVEHYLSDVCYTRAAGLFKNAAIASGLRSKIKSNFRLKELRNMKSGLPTTKSDNFPIPLVKQKGGQCTGFEISNHNSDFIIKIPFGRWQVKKEIDKYRPWEKFDFEQVRKSPKPISLLLSTQRRKRNKGWSKDEGTEAEIRKVMNGDYQTSYIEVTRGSKIGEKSTWMLNLSIDVPKIDKGVDPSIIGGIDVGVKSPLVCAINNAFSRYSISDNDLFHFNKKMFARRRILLKKNRHKRAGHGAKNKLKPITTLTEKSRRFRKKLIERWACEIADFFIKNKVGTVQMESLESMKRREDSYFNVRLRGFWPYAEMQSKIEFKLKQYGIVVRKVAPNNTSKTCSKCGHLNNYFNFEYRKKNKFPHFKCEKCNFKEDADYNAALNISNPKLKSTKGEP

SEQ ID NO: 2458 - protein, 726 aa, synthetic construct
SEVEFSHEYWMRHALTLAKRARDEREVPVGAVLVLNNRVIGEGWNRAIGLHDPTAHAEIMALRQGGLVMQNYRLTDATLYVTFEPCVMCAGAMIHSRIGRVVFGVRNSKRGAAGSLMNVLNYPGMNHCVEITEGILVDECAALLCDFYRMPRQVLNAQKKAQSGISSGGSSGGSGCSETPGASESVTPKSSGSSSAGSTKNTITKTLQLRIVRPYNSAEVEKIVTDEKNNREKIALEKNKDKVKEACSKHLKVAAYCTTQVERNACLFCKARKLDDKFYQKLRGQFPDAVFWQEIGEIFRQLQKQAAEIYNQSLVELYYEILIKGKGIANASSVEHYLSDVCYTRAAELFKNAAIASGLRNKIKSNFRLKELRNMRSGLPTTKSDNFPIPLVRQKGGQYTGFEISNHDGDFIIKIPFGRWQVKKEINKHRPWEKFDFEQVRKSPKPISLLLSTRRRKRNKGWSKDEGTEAEIRKVMNGDYQTSYIEVKRGSKIGEKSAWMLNLSIDVPKIDKGVDPSIIGGIDVGVKSPLVCAINNAFSRYSISDNDLFHFNKKVFARRRILLKKNRHKRAGHGAKNKLKPITILTEKSGRFRKKLIERWACEIADFFIKNKVGTVQMENLESMKRKEDSYFNIRLRGFWPYAEMQNKIEFKLKQYGIEVRKVAPNNTSKTCSKCGHLNDYFNFEYRKKNKFPHFKCEKCNFKENADYNAALNISNPKLKSTKEEP

SEQ ID NO: 2459 - protein, 726 aa, synthetic construct
SEVEFSHEYWMRHALSLAKRARDEREVPVGAVLVLNNRIIGEGWNRAIGLHDPTAHAEIMALRQGGLVMQNYRLIDATLYVTFEPCVMCAGAMVHSRIGRVVFGVRNSKRGAAGSLMNVLNYPGMNHRVVITEGILADECAALLCDFYRMPRQVFNARKKAQSSINPSGSSGGSSGSVTPGTSESATPESSGGGFGGSAKNTITKTLQLRIVRPYNSAEVEKIVADEKNNREKIALEKSKDKVKEACSKHLKVASYCTTQVERNACLFCKARKLDDKFYQKLRGQFPDAVFWQELGEIFRQLQKQAAEIYNQSLIELYYVIFIKGKGFANASSVEHYLSDVCYTRAAELFKNAAIASGLRGKVKSNFRLKELKNMKSGLPTTKSDNFPIPLVKQKGGQYTGFEISSHNDDFIIKIPFGRWQVKEEIDKYRPWEKFDFEQVRKSPKPISLLLSTQRRRKNKGWSKDEGTEAEIRRVMNGDYQTSYIEVKRGSKTGEKSAWMLNLSIDVPKIDKGVDPSIIGGIDVGVKSPLVCAINNAFSRYSISDNDLFRFNKKMFARRRILLGKNRHKRAGHGVKNKLKPITILTEKGGRFRKKLIERWACEIADFFIKNKVGTVQMENLESMKRKEDSYFNIRLRGFWPYAEMQNKIEFKLKQYGIEIRRVAPNNTSRTCSKCGHLNNYFNFEYRRKYKFPHFKCEKCNFKEDADYNAALNISNPKLKSTKEEP

SEQ ID NO: 2460 - protein, 726 aa, synthetic construct
SEVEFSHEYWMRHALTLAKRARDEREVPVGAVLVLNNRVIGEGWNRTTGLHDPTAHAEIMALRQGGLVMRNYRLTDATLYVTFEPCVMCAGAMIHSRIGRVVFGVRNSKHGAAGSLMNVLNYPGMNHRVEITEGILADECAGLLCDFYRMPRQVFSARKKAQSSIDPGGSSGGSSGGKAPGTSESATLESSGGSSGGSAKNSITKTLQLRIVRPYNSAEVEKIVADEKNNREKIALEKNKNKVKEACSKHLKVAAYCTTQVERNACLFCKARKLDDKFYQKLRGQFPDAVFWQEISEIFRQLQKQAAEIYNQSLIELYYEIFIKGKGFANASSVEHYLSDVCYTRAAELFKNAAIASGLRGKVKSNFRLKELKNMKSGLPTTKSDNFPIPLVKQKGGQYTGFEISSHNDDFIIKIPFGRWQVKKEIDKYRPWEKFDFEQVRKSPKPISLLLSTQRRKRNKGWSKDEGTEAEIRKVMNGDYQTSYIEVKRGSKIGEKSAWMLNLSIDVPKIDKGVDPSIIGGIDVGVKSPLVCAINNAFSRYSISDNDLFHFNKKVFARRRILLKKNRHRRAGHGAKNKLKPITILTEKSKRFRKKLIERWACEIADFFIKNKVGTVQMENLESMKRKEDSYFNIRLRGFWPYAEMQNKIEFKLKQYGIKIRKVAPNNTSRTCSKCGHLNNYFSFEYRKKNKFPHFKCEKCNFKEDADYNAALNISNPKLKGTKEEL

SEQ ID NO: 2461 - protein, 726 aa, synthetic construct
SEAEFSHEYWMRHALTLAKRARDEREVPVGAVLVLNNRVIGEGWNRAIGLHDPTAHAEIMALRQGGLVMQNYRLSDATLYVTFEPCVMCAGAMIHSRIGRVVFGVRNSKRGAAGSLMNVLNYPGMNHCVEITEGILVDECAALLCDFYRMPRQVFSARKKAQFSINSGGSSDGGSGSETPGTSESATQESSGDSSGGSAKNTITKTLKLRIVRPYNSAEVEKIVADEKNNREKIALEKNKDKVKEACSEHLKVAAYCTTQVERSACLFCKARKLDDKFYQKLRGQFPDAVSWQEIGEIFRQLQKQAAEIYNQSLIELYYEIFIKGKGFANASSVEHYLSDVCYTRAAELFKNAAIASGLRGKVKGNFRLKELKSMKSGLPTTKSDNFPIPLVKQKGGQYTGFEISSHNDDFIIKIPFGRWQVKKEIDKYRPWEKFDFEQVRKSPKPISLLLSTQRRKRNKGWSKDEGTEAEIRKVMNGDYQTSYIEVKRGSKIGEKSAWMLNLSIDVPKIDKGVDPSIIGGIDVGVRSPLVCAINNALSRYSISDNDLFHFNKKVFARRRILLKKNRHRRAGHGAKNKLKPITILTEKSKRFRKKLIERWACEIADFFIKNKVGIVQMENLESMKRREDSYFNIRLRGFWPYAEMQNKIEFKLKQYGIEIRKVAPNNTSKTCSRCGHLNNYFNFEHRKKNKFPRFKCEKCNFKENADYNAALNISNPKLKGTKEEP

SEQ ID NO: 2462 - protein, 726 aa, synthetic construct
SEVEFSHEYWMRHALTLAKRARDEREVPVGAILVLNNRVIGEGWNRAIGLHDPTAHAEIMALRQGGLVMQNYRLTDATLYATFEPCVMCAGAMIHSRIGRVVFGVRNSKHGAAGSLMNVLNYPGMNHRVEITEGILADECAGLLCDFYRMPRQVFSARKKAQSSINPGGSSGGSSGGKAPGTSESATLESSGGSSGGSAKNSITKTLKLRIVRPYNSAEVEKIVADEKNNREKTALEKNKDKVKEACSKHLKVAAYCTTQVERNACLFCKARKLDDKFYQKLRGQFPDAVFWQEVGEIFRQLQKQAAEIYNQSLIELYYEIFIKGKGFANASSVEHYLSDVCYTRAAELFKNAAIASGLRGKVKSNFRLRELKNMKSGLPTTKSDNFPIPLVKQKGGQYTGFEISNHNSDFIIKIPFGRWQVKKEINRYRPWEKFDFEQVRKSPKPISLLLSTQRRKRNKGWGKDEGTEAEIRKVMNGDYQTSYIEVKRGSRIGEKSAWMLSLSIDVPKIDRGVDPSIIGGIDVGVKSPLVCAINNALNRYSISDNDLFHFNKKMFARRRILLKKNRHRRAGHGAKNKLKPITVLTEKSKRFRKKLIERWACEIANFFIKNKVGTVQMENLESMKRKEDSYFNIRLRGFWPYAEMQNKIEFKLKQYGIGIRKVAPNNTSKTCSKCGHLNNYFNFEYRKKNKFPHFKCEKCNFKENADYNAALNICNPKLKSTKEEP

SEQ ID NO: 2463 - protein, 726 aa, synthetic construct
SEVEFSHEYWMRHALTLAKRARDEREVPVGAILVLNNRVIGEGWNRAIGLHDPTAHAEIMALRQGGLVMQNYRLIDATLYVTFEPCIMCAGAMVHSRIGRVVFGVRNSKRGAAGSLMNVLDYPGMGHRVEITEGILADECAALLCDFYCMPRQVFNAQKRTQSSINSGGSSGGSSGSETPGTSESATPESSGGGSSGSAKNTITKTLQLRIVRPYNSAEVEKIVADEKNNREKIALEKNKDKVKEACSKHLKVASYCTTQVERNACPFCKARKLDDKFYQKLRGQFPDAVFWQELGEILRQLQKQAAEIYNQSLIELYYEIFVKGKGIANTSRMEHYLSDVCYTRAAKLFKNAAIASGLRGKIKSNFRLKELKNMKSGLPTTKSDNFPIPLVKQKGGQYTGFEISSHNDDFIIKIPFGRWQVKKEIDKYRPWEKFDFEQVRRSPKPISLLLSTQRRKKNKGWSKDEGTEAEIRKVMNGDYQTSYIEVKRGSKIGEKSAWMLNLSIDVPKIDKGVDPSIIGGIDVGVKSPLVCAVNNALSRYSISDNDLFHFNKKMFARRRILLKKNRHRRAGHGAKNKLKPIAVLTEKSEGFRKKLIERWACEVADFFIKNKVGTVQMENLESMKRREDSYFNIRLRGFWPYAEMQNKIEFKLRQYGIEIRKVAPNNTSKTCSKCGHLNNYFDFEYRKKNKFPHFKCEKCNFKENADYNAALNISNPKLRSTKEEP

SEQ ID NO: 2464 - protein, 726 aa, synthetic construct; identical to SEQ ID NO: 684

SEQ ID NO: 2465 - protein, 726 aa, synthetic construct
SEVEFSHEYWMRHALTLAKRARDEREVPVGAVLVLNNRVIGEGWNRAIGLHDPTAHAEIMALRQGGLVMQNYRLIDATLYVTFEPCVMCAGAMVHSRIGRVVFGVRNSKRGAAGSLMNVLDYPGMGHRVEITEGILADECAALLCDFYCMPRQVFNAQKRAQSSINSGGLSGGSSGSDTPGTSESATPESSGGSSGGSAKNTITKTLQLRIVRPYNSAEVEKIVADEKNNREKIALEKNKDKVREACSKHLKVASYCTTQVERNACLFCKARKLDDRFYQKLRGQFPDAVFWQELGEIFRQLQKQAAEIYNQSLIELYYEIFIKGKGLANASSVEHYLSDVCYTRAAELFKNAAIASGLRGKVKSNFKLKELKSMKSGLPTTKSDNFPIPLVKQKGGQYTGFEISSHNEDFIIKVPFGRWQVKKEIDKYRPWEKFDFEQVRKSPKPISLLLSTQRRRRNKGWSKDEGTEAEIRKVMNGDYQTSYIEVKRGSKIGEKSAWMLNLSIDVPKIDKGVDPSIVGGIDVGVKSPLVCAINNALSRYSISDNDLFHFNKKMFARRRILLKKNRHRRAGHGAKNKLRPITILTEKSKRFRRKLIERWACEIADFFIKNKVGTVQMENLESMKRKEDSYFNIRLRGFWPYAEMQNKIEFKLKQYGIEIRKVAPNNTSKTCSKCGHLNNYFNFEYRKKNKFPHFKCEKCNFKESADYNAALNISNPKLKSTKGEP

SEQ ID NO: 2466 - protein, 726 aa, synthetic construct
SEVGFSHEYWMRHALTLAKRARDEREVPVGAVLVLNNRVIGEGWNRAIGLHDPTAHAEIMALRQGGLVMQNYRLTDATLYVTFEPCVMCAGAMIHSRIGRVVFGVRNSKRGAAGSLMNVLNYPGMNHCVEITEGILVDECAALLCDFYRMPRQVLNAQKKAQSSISPGGSSGGSSGSGTPGASGSVTPKSSGGSSAGSTKDTITKTLKLRIVRPYNSAEVEKIVADEKDSREKIALEKNKDMVKEACSKHLKVASYCTTQVERNACLFCKARKLDDKFYQKLRGQFPDAVFWQELGGIFRQLQKQAAEIYNQSLIELYYEIFIKGKGITNASRVEHYLSDVCYTRAAELFKNAAIASGLRSKVRSNFRLKELKNMKSGLPTTKSDNFPIPLVKQKGGQYTGFEISSHNSDFIIKIPFGRWQEKEEIGKYRPWEKFDFEQVRRSPKPISLLLSTQRRKKNKGWGKDEGTEAEIRRVMNGDYQTSYIEVKRGSKIGEKSAWMLNLSIDVPKIDKGVDPSIIGGIDVGVKSPLVCAINNAFSRYSISDNDLFHFNKKMFARRRILLKKNRRRRAGHGAKNKLKPITILTEKSVRFRKKLIERWACEIADFFIKNKVGTVQMENLESMKRKEDSYFNIRLRGFWPYAEMQNKIEFKLKQYGIEIRKVAPNNTSRTCSKCGHLNNYFNFEYRKKNKFPHFKCEKCNFKEDADYNAALNISNPKLKSTKEEP

SEQ ID NO: 2467 - protein, 726 aa, synthetic construct
SEVEFSHEYWMRHALTLAKRARDEREVPVGAILVLNNRVIGEGWNRAIGLHDPTAHAEIMALRQGGLVMQNYRLIDATLYVTFEPCVMCAGAMIHSRIGRVVFGVRNNKHGAAGSLVNVLNYPGMNHRVEITEGILVDECAALLCDFYRMPRQVFNAQKRAQSSINSGGSSGGSSGSETPSTSESATPESSGGSSGGSAKNTITKTLTLRIVRPYNSAEVEKIVADEKNNREKIALEKNKDKVKEACSKHLKVAAYCTTQVERNACLFCKARKLDDKFYQKLRDQFPDAVFWQEIGEIFRQLQKQAAEIYNQSLIELYYEIFIKGKGFANASSVEHYLSDVCYTRAAELFKNAAIASGLRGKVKSNFRLKELKNMKSGLPTTKSDNFPIPLVKQKGGQYTGFEISSHDDDFVIKIPFGRWQVKKEIDKYRPWEKFDFEQVRKSPKPISLLLSTQRRKRNKGWSKDGGTEAEIRKVMNGDYQTSYIEVKRGSRIGEKSAWMLSLSIDVPKIDRGVDPSIIGGIDVGVKSPLVCAINNALSRYSISDNDLFHFNKKMFARRRILLKKNRHRRAGHGARNKLKPITVLTEKSKRFRKKLIERWACEIANFFIKNKVGTVQMENLESMKRREDSYFNIRLRGLWPYAEMQNKIEFKLKQYGIKIRKVAPNNTSKTCSKCGHLNNYFNFEYRKRNKFPHFKCEKCNFKENADYNAALNISNPKLKGTKEEP

SEQ ID NO: 2468 - protein, 726 aa, synthetic construct
SEVEFSHEYWMRHALTLAKRARDEREVPVGAVLVLNNRVIGEGWNRAIGLHDPTAHAEIMALRQGGLVMQNYRLVNATLYVTFEPCVMCAGAMIHSRIGRVAFGVRNSKRGAAGSLMNVLSYPGMNHRVEITEGILAGECAALLCDFYRMPRQVFNARKKAQSNISSGGSSGGSSGSETPDASGSVTPKSSGGSSAGSTKGTITKTLKLRIVRPYNSAEVEKIVADEKNNREKIALEENKDKVKEACSEHLKVAAYCTTQVERNACPFCKARKLDDKFYQKLRGQFPDAVFWQELGEILRQLQKQAAEIYNQSLIELYYEIFIKGRGFANASSVEHYLSDVCYTRAAGLFKNAAIASGLRGKVKSNFRPKELKNMKSGLPTTKSDNFPIPLVKQKGGQYTGFEICNHNDDFIIKIPFGRWQVKKEIDKYRPWEKFDFEQVRKSPKPISLLLSTQRRKRNKGWSKDEGTEAEIRKVMNGDYQTSYIEVKRGSKIGEKSAWMLNLSIDVPRIDKGVDPSIIGGIDVGVKSPLVCAINNAFSRYSISDNDLFRFNKKMFARRRILLGKNRHKRAGHGVKNKLKPITILTEKSGRFRKKLIERWACEIADFFVKNKVGTVQMENLESMKRKEDSYFNIRLRGFWPYAEMQNKIEFKLKQYGIEVRKVAPNNTSKTCSKCGHLNNYFNFEYRKKNKFPPFKCEKCNFKENADYNAALNISNPKLKGTKEEP

SEQ ID NO: 2469 - protein, 726 aa, synthetic construct
SEDEFSHEYWMRHALTLAKRARDGREVPVGAVLVLNNRVIGEGWNRAIGLHDPTAHAEIMALRQGGLVMQNYRLIDATLYVTFEPCVMCAGAMVHSRIGRVVFGVRNSKRGAAGSLMNVLDYPGMGHRVEITEGILADECAALLCDFYCMSRQVFNAQKRAQPSINSGGSSGGSSGSETPGTSESATPESSGGGSSGSAKNTITKTLRLRIVRPYNSAEVEKIVADEKNNREKIALEKNKGKVKEACSKHLKVAAYCTTQVERNACLFCKARKLDDKFYQKLRGQFPDAVFWQEIGEIFRQLQKQAAEIYNQSLIELYYEIFIKGRGFANASSVEHYLSDVCYTRAAELFKNAAIASGLRSKVRSNFRLKELKNMKSGLPTTKSDNFPIPLVKQKGGQYTGFEISSHNSDFIIKIPFGRWQVKKEINKFRPWEKFDFEQVRKSPKPISLLLSTQRRKKNKGWSKDEGTEAEIRRVMNGDYQTSYIEVKRGSKIGEKSAWMLNLSIDVPKIDKGVDPSIIGGIDVGVKSPLVCAINNSSSRYSISDNDLFRFNKKMFARRRILLKKNRHKRAGHGAKNKLKPISILTEKSKRFRKKLIERWACEIADFFIKNKVGTVQMENLESMKRKEDSYFNIRLRGFWPYAEMQNKIEFKLKQYGIEIRKVAPNNTSKTCSKCGHLNNYFNFEYRKKNKFPHFKCEKCNFKEDADYNAALNISNPKLKSTKEEP

SEQ ID NO: 2470 - protein, 726 aa, synthetic construct
SEDEFSHEYWMRHALTLAKRARDEREVPVGAILVLNNRVIGEGWNRAIGLHDPTAHAEIMALRQGGLVMQNYRLIDATLYVTFEPCVMCAGAMIHSRIGRVVFGVRNNKHGAAGSLVNVLNYPGMNHRVEITEGILADECAALLCDFYRMPRQVFNARKKAQSSINPGGSSGGSSGSETPGTSESPTPESSGGSSGGSAKNTITKTLKLRIVRPYNSAEVEKIVADEKNNREKIALEKNKDKVKEACSKHLKVAAYCTTQVERNACLFCKARRLDDKFYQKLRGQFPDAVFWQEIGEIFRQLQKQAAEIYNQSLIELYYEIFIKGKGIANASSVEHYLSDVCYTRAAELFKNAAIASGLRNKVKSNFRLKELRSMKSGLPTTKSDNFPIPLVRQKGGQYTGFGISNHNGDFIIKIPFGRWQVKKEINKHRPWEKFDFEQVRKSPKPISLLLSTQRRKRNKGWSKDEGTEAEIRKVMNGDYQTSYIEVKRGSKIGEKGAWMLNLSIDVPKIDKGVDPSIIGGIDVGVKSPLVCAINNALSRYSISDNDLFHFNKKMFARRRILLRKNRHKRAGHGARNKLKPITVLTEKSERFRRKLIERWACEIANFFIKNKVGTVQMENLESMKRREDSYFNIRLRGFWPYAEMQNKIEFKLKQYGIEIRKVAPNNTSKTCSKCGHLNNYFNFEFRKKNKFPHFKCEKCNFKEDADYNAALNISNPKLKSTKEEP

SEQ ID NO: 2471 - protein, 726 aa, synthetic construct
SVVEFSHEYWMRHALTLAKRARDEREVPVGAVLVLNNRVIGEGWNRAIGLHDPTAHAEIMALRQGGLVTQNYRLIDATLYVTFEPCVMCAGAMVHSRIGRVVFGVRNSKRGAAGSLMNVLDYPGMGHRVEITEGILADECAALLCDFYCMPRQVFNAQKRAQSSINSGGSSGGSSGSETPGTSESATPESSGGGSSGSAKNAITKTLQLRIVRPYNSAEVEKIVADEKNNREKIALEKNKDKVKEACSKHLKVASYCTTQVERNACPFCKARKLDDKFYQKLRGQFPDAVFWQELGEILRQLQKQAAEIYNQSLIELYYEIFIRGRGFANAGSVEHYLSDVCYTRAAELFKNAAIASGLRGKVKSNFRLKELKNMKSGLPTTKSDNFPIPLVKQKGGQYTGFEISSHDDDFIIRIPFGRWQVKKEIDKFRPWEKFDFEQVRKSPKPISLLLSTQRRKRNKGWSKDEGTEAEIRKVMSGDYQTSYIEVKRGSKTGEKSAWMLNLSIDVPKIDKGVDPSIIGGIDVGVKSPLVCAINNTFSRYSISDNDLFRFNKKMFARRRILLKKNRHKRAGHGAKNKLKPISILTGKSERFRKKLIERWACEIADFFIKNKVGTVQMENLESMKRKEDSYFNIRLRGFWPYAEMQNKIEFKLKQYGIEIRKVAPNNTSKTCSKCGHLNNYFSFEYRKKNKFPHFKCEKCNFKENADYNAALNISNPKLMSTKEEP

SEQ ID NO: 2472 - protein, 726 aa, synthetic construct
SEVEFSHEYWMRHALTLAKRARDEREVPVGAILVLNNRVIGEGWNRAIGLHDPTAHAEIMALRQGGLVMQNYRLIDATLYVTFEPCAMCAGAMVHSRIGRVVFGVRNSKRGAAGSLMNVLNYPGMDHRVEITGGILADECAALLCDFYRMPRRVFSAQKKARSNINSGGSSGGSSGSETLGTSESVTPESSGGSSGGPAKNTITKTLKLRIVRPYNSAEVEKIVADEKNNREKTALEKNKDKVKEACSKHLKVAAYCTTQVERNACLFCKARKLDDKFYQKLRGQFPDAVFWQEVGEIFRQLQKQAAEIYNQSLIELYYEIFIKGKGITNASRVEHYLSDVCYTRAAELFKNAAIASGLRSKVRSNFRLKELKNMKSGLPTTKSDNFPIPLVKQKGGQYTGFEISSHNSDFIIKIPFGRWQVKEEIDKYRPWEKYDFEQVRKSPKPISLLLSTQRRKRNKGWSKDEGTEAEIRKVMNGDYQTSYIEVKRGSKTGEKSAWMLNLSIDVPKIDKGVDPSIIGGIDVGVKSPLVCAINNAFSRYSISDNDLFRFNKKMFARRRILLRKNRHKRAGHGAKNKLKPISILTGKSERFRKKLIERWACEIADFFIKNRVGTVQMENLESMKRKEDSYFNIRLRGFWPYAEMQNKIEFKLKQYGIEIRKVAPNNTSKTCSKCGHLNNYFNFEYRKKNKFPHFKCEKCNFKENADYNAALNISNPKLKSTKEEP

SEQ ID NO: 2473 - protein, 726 aa, synthetic construct
GEVEFSHEYWMRHALTLARRARDGREVPVGAVLVLNNRVIGEGWNRAIGLHDPTAHAEIMALRQGGLVMQNYRLIDATLYVTFEPCVMCAGAMVHSRIGRVVFGVRNSKRGAAGSLMNVLDYPGMGHRVEITEGILADECAALLCDFYCMPRQVFNAQKRAQSSINSGGSSGGSSGSETPGTSESVTPKSSGGSSAGSTKNTITKTLKLRIVRPYNSAEVEKIVADEKNSREKIALERNKDKVKEACSEHLEVAAYCTTQVERNACLFCKARKLDDKFYQKLRSQFPDAVFWQELGEIFRQLQKQAAEIYNQSLIELYYEIFIKGKGFANAGSVEHYLSDVCYTRAAELFKNAAIASGLRGKVKSNFRLKELKNMKSGLPTTKSDNFPIPLVKQKGGQYTGFEISSHNDDFIIKIPFGKWQVKKEIDKYRPWEKFDFEQVRKSPKPISLLLSTQRRKRNKGWSKDEGTEAEIRKVMNGDYQTSYIEVKRGSRTGEKSAWMLSLSIDVPKIDKGVDPSIIGGIDVGVKSPLVCAINNAFNRYSISDNNLFHFNKKMFARRRILLKKNRHKRAGHGAKNKLKPISILTEKSERFRKKLIERWACEIADFFIRNKVGTVQMENLEGMKRKEDSYFNVRLRGFWPYAEMQNKIEFKLKQYGIEVRKVAPNNTSKTCSKCGHLNNYFNFEYRKKNKFPHFKCEKCNFKENADYNAALNISNPKLKSTKEEP

SEQ ID NO: 2474 - protein, 726 aa, synthetic construct
SEVEFSHEYWMRHALTLAKRARDEREVPVGAVLVLNNRVIGEGWNRAIGLHDPTAHAEIMALRQGGLAMQNYRLVDATLYVTFEPCVLCAGAMVHSRIGRVVFGVRNSKRGAAGSLMNVLNHPGMNHRVEITGGILADECAALLCDFYRMPRQVFNVQKKARSNINSGGSSGGSSGNETPGASESATPKSSSGSSAGSTKNTITKTLKLRIVRPYNSAEVEKIVADEKNNRERIALEKNKDKVKEACSKHLKVAAYCTTQVERNACLFCKARKLDDKFYQKLRGQFPDAVFWQETGEIFRQLQRQAAEIYNQSLIELYYEIFIKGKGFANASSVEHYLSDVCYTRAAELFKNAAIASGLRGKVKSNFRLKELKNMKSGLPTTKSDNFPIPLVKQKGGQCTGFEISNHNSDFIIKIPFGRWQVKKEIDKYRPWEKFDFEQVRKSPKPISLLLSTQRRKRNKGWSKDEGTEAEIRKVMNGDYQTSYIEVKRGSKIGEKGAWMLNLSIDVPKIDKGVDPSIIGGIDVGVKSPLVCAINNAFSRYSISDNDLFRFNKKMFARRRILLKKNRHRRAGHGAKNKLKPISILTGKSGRFRKKLIERWACEIADFFIKNKVGTVQMENLESMKRKEDSYFNIRLRGFWPYAEMQNKIEFKLKQYGIEIRKVAPNNTSKTCSKCGHLNNYFNFEYRKKNKFPHFKCEKCNFKENADYNAALNISNPKLKSTKEEP

SEQ ID NO: 2475 - protein, 726 aa, synthetic construct
GEAEFSHEYWMRRALTLAKRARDEREVPVGAILVLNNRVIGEGWNRAIGLHDPTAHAEITALRQGGLVMQNYRLIDATLYVTFEPCVMCAGAMVHSRIGRVVFGVRNSKRGAAGSLMNVLDYPGMGHRVEITEGILADECAALLCDFYCMPRRVFNAQKRAQSSINPGGSSGGSSGSETPGTSESATPESSGGSSGGSAKNTITKTLKLRIVRPYNSAEVEKIVADEKNDREKIALEKNKDKVKEACSEHLKVAAYCTTQVERSACLFCKARKLDDKFYQKLRGQFPDAVFWQELGEILRQLQKQAAEIYNQSLIELYYEIFIKGKGFTNASGVEHYLSDVCYTRAAELFKNAAIASGLRGKVKSNFRLKELKNMKSGLPTTKSDNFPIPLVKQKGGQYAGFEISSHNDDFIIKIPFGRWQVKKEIDKYRPWEKFDFEQVRKSPKPISLLLSTRRRKRNKGWSKDEGTEAEIRKVMNGDYQTSYIEVKRGSKIGEKSAWMLNLSIDVPKIDKGVDPSIIGGIDVGVKSPLVCAVNNAFSRYSISDNDLFRFNKKMFARRRILLGKNRHKRAGHGVKNKLKPITILTEKSGRFRKKLIERWACEIADFFVKNMVGTVQMENLESMKRKEDSYFNIRLRGFWPYAEMQNKIEFKLKQYGIEVRKVAPNNTSKTCSRCGHLNNYFNFEYRKKNKFPHFKCEKCNFKEDADYNAALNISNPKLKSPKEEP

SEQ ID NO: 2476 - protein, 726 aa, synthetic construct; identical to SEQ ID NO: 684

SEQ ID NO: 2477 - protein, 726 aa, synthetic construct
SEVEFSHEYWMRHALTLAKRARDEREVPVGAVLVLNNRVIGEGWNRAIGLHDPTAHAEIMALRQGGLVMQNYRLIDATLYVTFEPCVMCAGAMIHSRIGRVVFGVRNNKRGAAGSLMNVLNYPGMNHRVEITEGILADECAALLCDFYRMPHQVLNAQKKARSCINPGGSSGGSSGSETPGTSESATPESSGGSSGGSAKNTITKALKLRIVRPYNSAEVEKIVADEKNNREKIALEKNKDKVKEACSKHLKVAAYCTTQVERNACLFCKARKLDDKFYQKLRGQFPDAVFWQEIGEIFRQLQKQAAEIYNQSLVELYYEIFIKGKGIANASSVGHYLSDVCYTRAAELFKNAAIASGLRNKIKSNFRLKELKNMKSGLPTTKSDNFPIPLVKQKGGQYTGFEISSHNDDFIIKIPFGRWQVKKEIDKYRPWEKFDFEQVRKSPKPISLLLSTQRRKRNKGWSKDEGTEAEIRKVMNGDYQTSYIEVKRGSKIGEKSAWMLNLSIDVPKINKGVDPSIIGGIDVGVKSPLVCAINNAFSRYSISDNDLFHFNKKMFARRRILLKKNRHKRAGHGAKNKLKPISILTEKSKRFRKKLIERWACEIADFFIKNKVGTVQMENLESMKRKEDSYFNIRLRGFWPYAEMQNKIEFKLKQYGIEIRRVAPNNTSKTCSKCGHLNNYFNFEYRKKNKFPHFKCEKCNFKENADYNAALNISNPKLKSTKEEP

SEQ ID NO: 2478 - protein, 726 aa, synthetic construct
SEDEFSHEYWMRHALTLAKRARDGREVPVGAVLVLNNRVIGEGWNRAIGLHDPTAHAEIMALRQGGLVMQNYRLTDATLYVTFEPCVMCAGAMIHSRIGRVVFGVRNSKHGAAGSLVNVLNYPGMNHRVEITEGILADECAALLCDFYRMPRQVFNARKKAQSSTNPGGSSGGSSGSETPGTSESATLENSGGSSGGSAKNTITKTLKLRIVRPYNNAEVERIVADEKNNREKIALEKNKDKVKEACSEHLKVAAYCTTQVERNACLFCKARRLDDKFYQKLRGQFPDAVFWQETGEIFRQLQRQAAEIYNQSLIELYYELFIKGKGFANASSVEHYLSDVCYTRAAELFKNAAIASGLRGKVKSNFRLKELKNMKSGLPTTKSDNFPIPLVKQKGGQYTGFEISSHNDDFIIKIPFGRWQVKKEIDKYRPWEKFDFEQVRKSPKPISLLLSTQRRRRNKGWSKDEGTEAEIRKVMNGDYQTSYIEVKRGSKIGEKSAWMLSLSIDVPKIDKGVDPSIIGGIDVGVKSPLVCAINNAFSRYSISDNDLFRFNKKMFARRRILLKRNRHQRAGHGAKNKLKPITILTEKSGRFRKKLIERWACEIADFFIKNKVGTVQMENLESMKRKEDSYFNIRLRGFWPYAEMQNKIEFKLKQYGIKIRKVAPNNTSKTCSKCGHLNNYFSFEYRKKNKFPHFKCEKCNFKENADYNAALNISNPKLMSTKEEP

SEQ ID NO: 2479 - protein, 726 aa, synthetic construct
SEDEFSHEYWMRHALTLAKRARDGREVPVGAVLVLNNRVIGEGWNRAIGLHDPTAHAEIMALRQGGLVMQNYRLIDATLYVTFEPCVMCAGAMVHSRIGRVVFGVRNSKRGAAGSLMNVLDYPGMGHRVEITEGILADECAALLCDFYCMPRQVFNAQKRAQSSINSGGSSGGSSGSETPGTSESATPESSGGGSSGSAKSTITKTLQLRIVRPYNSAEVEKIVADEKNNREKIALEKNKDKVKEACSKHLKVASYCTTQVERNACPFCKARKLDDKFYQKLRGQFPDAVFWQELGEILRQLQKQAAEIYNQSLIELYYEIFIKGRGFANASSVEHYLSDVCYTRAAELFKNAAIASGLRGKVKSNFRLKELKNMKSGLPTTKSDNFPIPLVKQKGGQYTGFEISSHNDDFIIKIPFGRWQVKKEIDKYRPWEKFDFEQVRKSPKPISLLLSTQRRKRNKGWSKDEGTEAEIRKVMNGDYQTSYIEVKRGSKIGEKSAWMLNLSIDVPKIDKGVDPSTIGGIDVGVKSPLVCAINNAFSRYSIGDNDLFHYNKKMFARRRILLKKNRHKRAGHGAENKLKPISILTEKSKKFRKKLIERWACEIADFFIKNKVGTVQMENLESMKRKEDSYFNIRLRGFWPYAEMQNKIEFKLKQYGIEIRKVAPNNTSRTCSKCGHLNNYFNFEYRMKNKFPLFKCEKCNFKEDADYNAALNISNPKLKSTKEEP

SEQ ID NO: 2480 - protein, 726 aa, synthetic construct
SEVEFSHEYWMRHALTLAKRARDEREVPVGAVLVLNDRVIGEGWNRMTGLHDPTAHAEIMALRQGGLVMQNHRLVDATLYVTFEPCVMCAGAMIHSRIGRVVFGVRNSKRGAAGSLTNVLNYPGMNHRVEITEGILVDECAALLCDFYRMPHQVFNAQKKAQSTINSGGSSGGSSGSETPGTSESPTPESSGGSPGGSARNTITKTLKLRIVRPYNSAEVEKIVADEKNSREKIALEKNKDKVKEACSEHLKVAAYCTTQVERNACLFCKARKLDDGFYQKLRGQFPDAVFWQEIGEIFRQLQKQAAEIYNQSLIELYYEIFIKGKGFANASSVEHYLSDVCYTRAAELFKNAAIASGLRGKVKSNFRLKELKNMKSGLPTTKSDNFPIPLVKQKGGQYTGFEISSHNDDLIVKIPFGRWQVKKEIDRYRPWEKFDFEQVRKSPKPISLLLSTQRRKRNKGWSKDEGTEAEIKKVMNGDYQISYIEVKRGSKIGEKSAWTLNLSVDVPKIDKGVDPSIIGGIDVGVKSPLVCAINNALSRYSISDNDLFHFNKKVFARRRILLKKNRHRRAGHGAKNKLKPITILTEKSKRFRKKLIERWACEIADFFIKNKVGIVQMENLESMKRKEDSYFNIRLRGLWPYAEMQNKIEFKLKQYGIEIRKVAPNNTSKTCSKCGHLNNYFNFEYRKTNKFPYFKCEKCNFKEDADYNAALNISNPKLKSTKEEP

SEQ ID NO: 2481 - protein, 726 aa, synthetic construct
SEVEFSHEYWMRHALTLAKRARDGREVPVGAVLVLNNRVIGEGWNRAIGLHDPTAHAEIMALRQGGLVMQNYRLTDATLYVTFEPCVMCAGAMIHSRIGRVVFGVRNSKRGAAGSLMNVLNHPGMNHRVEITEGILVDECAALLCDFYRMPCQVLNAQKKAQSSISSGGSSGGSSGGDTLGASESVTPKSSVGSSASSTKNTITKTLKLRIVRPYNSAEVEKIVADEKNNREKIALEKNEDKVKEACSKHLKVAAYCTTQVERNACLFCKARKLDDKFYQELRGQFPGAVFWQEIGEIFRQLQKQAAEVYNQSLIELYYEIFIKGRGFANASSVEHYLSDVCYTRAAELFKNAAIASGLRGKVKSNFRLKELRNMKSGLPTTKSDNFPIPLVKQKGGQYTGFEISSHNDDFIIKIPFGRWQVKKEIDRYRPWEKFDFEQVRKSPKPISLLLSTQRRKRNKGWSKDEGTEAEIRKVMNGDYQTSYIEVKRGSKIGEKSAWMLSLSIDVPKIDKGVDPSTIGGIDVGVKSPLVCAINNAFCRYSISDNDLFHFNKKMFARRRILLKKSRHKRAGHGAKNKLKPISILTEKSKRFRKKLIERWACEIADFFVKNKVGTVQMENLESMKRKEDSYFNIRLRGFWPYAEMQNKIEFKLKQYGIEIRKVAPNNTSKTCSKCGHLNNYFNFEYRRKNKFPHFKCEKCNFKENADYNAALNISNPKLKSTKEEP

SEQ ID NO: 2482 - protein, 726 aa, synthetic construct
SEVEFSHGYWMRHALTLAKRARDEREVPVGAVLVLNNRVIGEGWNRAIGLHDPTAHAEIMALRQGGLVMQNYRLTDATLYVTFEPCVMCAGAMIHSRIGRVVFGVRNSKRGAAGSLMNVLNYPGMNHCVEITEGILVDECAALLCDFYRMPRQVLSAQKKAQSSISSGGPSGGSSCSETPGASESVTPKSSGGSSTGSTKNTITKTLKLRIVRPYNSAEVEKIVADEKNNREKIALEKNKDKVKEACSEHLKVAAYCTTQVERNACLFCKARKLDDKFYQKLRGQFPDAVFWQEIGEIFRQLQKQAAEIYNQSLVELYYEILIKGKGIANASSVEHYLSDVCYTRAAGLFKNAAIASGLRNKIKSNFRLKELRNMKSGLPTTKSDNFPIPLVKQKGGQYTGFEISNHDGDFIIKIPFGRWQVKREINKHRPWEKFDFEQVRKSPKPISLLLSTQRRKGNKGWSKDEGTEAEIRKVMNGDYQTSYIEVKRGSKIGEKSAWMLNLSIDVPKIDKGVDPSIIGGIDVGVKSPLVCAINNAFSRYSISDNDLFRFNKKVFARRRILLKKNRHKRAGHGTKNKLKPITILTEKSGRFRKKLIERWACEIANFFIKNKVGTVQMEYLESMKRKEDSYFNIRLRGFWPYAEMQNKIEFKLKQYGIKIRKVAPNNTSKTCSKCGHLNDYFSFEYRKRNKFPHFKCEKCNFKENADYNAALNISNPKLKGTKEEP

SEQ ID NO: 2483 - protein, 726 aa, synthetic construct; identical to SEQ ID NO: 684

SEQ ID NO: 2484 - protein, 726 aa, synthetic construct
SEVEFSHEYWMRHALTLAKRARDEREVPVGAVLVLNNRVIGEGWNRAIGLHDPTAHAEIMALRQGGLVLQNYRLVDATLYVTFEPCVLCAGAMVHSRIGRVVFGARNSKRGAAGSLMNILNYPGMNHRVEITEGILADECAALLCDFYHMPRQVFNAQKKAQSSINSGGSSGGSSGSETPSTSECATPKSSGGSSAGSTKNTITKTLKLRIVRPYNGAEVEKIVADEKNSREKIALERNKDKVKEACSKHLEVAAYCTTQVERSACLFCKARKLDDKFYQKLRGQFPDAVFWQEIGEIFRQLQKQAAEIYNQSLIELYYEIFIKGKGFANASSVEHYLSDVCYTRAAELFKNAAIASGLRGKVKSNFRLKELKNMKSGLPTTKSDNFPIPLVKQKGGQYTGFEISSHNDDFIIKIPFGRWQVKKEIDKYRPWEKFDFEQVRKSPKPISLLLSIQRRKRNKGWSKDEGTEAEIRKVMNGDYQTSYIEVKRGSKIGEKSAWMLNLSIDVPKIDKGVDPSIIGGIDVGVKSPLVCAINNAFCRYSISDNDLFHFNKKMFARRRILLKKSRHKRAGHGAKNKLKPISILTEKSKRFRKKLIERWACEIADFFIKNKVGTVQMENLESMKRKEDSYFNIRLRGFWPYAEMQNKIEFKLKQYGIKIRKVAPNNTSKTCSKCGHLNNYFNFEYRKKNKFPHFKCEKCNFKENADYNAALNISNPKLKSTKEEP

SEQ ID NO: 2485 - protein, 726 aa, synthetic construct
SEVEFSHEYWMRHALTLAKRARDEREVPVGAVLVLNNRVIGGGWNRAIGLHDPTAHAEIMALRQGGLVMQNYRLIDATLYVTFEPCVMCAGAMIHSRIGRVVFGVRNSKRGAAGSLMNVLNYPGMNHRVEITEGILAGECAALLCDFYRMPRQVFNAQKKAQSTINSGGSSGGSSSSETPGTSGSATPEGSGGSSGGSAKNTITKTLKLRIVRPYNSAEVEKIVADEKNNREKIALEKNKDKVKEACSKHLKVATYCTTQVERNACLFCKARKLDDKFYQKLRGQFPDAVFWQEIGEIFRQLQKQAAEIYNQSLIELYYEIFIKGKGITNASRVEHYLSDVCYTRAAELFKNAAIASGLRSKVRSNFRLKELKNMKSGLPTTKSDNFPIPLVKQKGGQYTGFEISSHNSDFIIKIPFGRWRVKEEIDKYRPWEKFDFEQVRKSPKPISLLLSTLRRKRNKGWSKDEGTEAEIRKVMNGDYQTSYIEVKRGSKIGEKSAWMLNLSIDVPKIDKGVDPSIIGGIDVGVRSPLVCAINNAFSRYSISDNDLFRFNKKMFARRRILLKKNRHKRAGHGAKNKLKPITILTEKSRRFRKKLIERWACEIADFFIKNKVGTVQMESLESMKRKEDSYFNIRLRGFWPYAEMQNRIEFKLKQYGIEIRKVAPNNTSKTCSKCGHLNNYFNFEYRKKNKFPHFKCERCSFKENADYNAALNISNPKLKSTKEEP

SEQ ID NO: 2486 - protein, 726 aa, synthetic construct
SEIEFSHEYWMRHALTLARRARDEREVPVGAILVLNNRVIGEGWNRAIGLHDPTAHAEIMALRQGGLVMQNYRLTDATLYVTFEPCVMCAGAMIHSRIGRVVFGVRNSKHGAAGSLVNVLNYPGMNHRVEITEGVLADECAALLCDFYRMPRQVFNARKKAQSSINPGGSSGGSSGSETPGTSESATLENSGGSSGGSAKNTITKTLKLRIVRPYNSAEVEKIVVDEKNNREKVALEKNKDEVKEACSEHLKVAAYCTTQVERSACLFCKARKLDDKFYQKLRGQFPDAVFWQEIGEIFRQLQKQAAEIYNQSLIELYYEIFIKGKGFANASSVEHYLSDVCYTRAAELFKNAAIASGLRGKVKSNFRLKELKNMKSGLPTTKSDNFPIPLVKQKGGQYTGFEISSHNDDFIIKIPFGRWQVKKEIDKYRPWEKFDFEQVRKSPKPISLLLSTQRRKRNKGWSKDEGTEAEIRKVMNGDYQTSYIEVKRGSKIGEKNAWMLNLSIDVPKIDKGVDPSIIGGIDVGVKSPLVCAINNAFSRYSISDNDLFRFNKKMFARRRILLKKNRHKRAGHGAKNKLKPISILTGKSERFRKKLIERWACEIADFFIKNKVGTVQMENLESMKRREDSYFNIRLRGFWPYAEMQNKIEFKLKQYGIEIRKVAPNNTSKTCSRCGHLNNYFNFEYRKKSKFPHFKCEKCNFKENADYNAALNISNPKLKSTKEEP

SEQ ID NO: 2487 - protein, 726 aa, synthetic construct
SEVEFSHEYWMRHALTLAKRARDEREVPVGAVLVLNNRVIGVGWNRAIGLHDPTAHAEIMALRQGGLVMQNYRLTDATLYVTFEPCVMCAGAMVHSRIGRVVFGVRNSKRGAAGSLMNVLNYPSMSHCVEITEGILVDECAALLCDFYRMPRQVFGARRKAQSSINPGGSSGGSSSSETPGTSESPTPESPGGSSGGSAKNTITKTLQLRIVRPYNSAEVEKIVTDEKNNREKIALEKNKDKVKEACSKHLKMASYCTTQVERNACLFCKARKLDDKFYQKLRGQFPDAVFWQEIGEIFRQLQKQAAEIYNQSLVELYYEVFVKGKGIANTSSVEHYLSDVCYTRAAELFKNAAIASGLRNKIKSNFRLKELRNMKSGLPTTKSDNFPIPLVKQKGGQYTGFEISSHNDDFIIKIPFGRWQAKKEIDRYRPWEKFDFEQVRKSPKPISLLLSTRRRKRNKGWSKDEGTEAEIRRVMNGDYQTSYIEVKRGSKIGEKSAWMLSLSIDVPKIDKGVDPRIIGGIDVGVKSPLVCAINNVPSRYSISDNDLFHFNKKMFARRRILLKKNRHKRAGHGAKNKLKPITILTEKSGRFRKKLIERWACEIANFFIKNKVGTVQMENLESMKRKEDSYFNIRLRGFWPYAEMQNKIELKLKQYGIKIRKVAPNNTSKTCSKCGHLNDYFNFEYRKKNKFPHFKCEKCNFKEDADYNAALNICNPKLKGTKEEP

SEQ ID NO: 2488 - protein, 726 aa, synthetic construct
SEVEFSHEYWMRHALSLAKRARDEREVPVGAVLVLNNRVIGEGWNRAIGLHDPTAHAEIMALRQGGLVMQNYRLIDATLYVTFEPCVMCAGAMIHSRIGRVVFGVRNNKRGAAGSLMNVLNYPGMNHRVEITEGILADECAALLCDFYCMPRQVLNAQKKARSCINSGGSSGGSSGSETPGTSESATPESSGGSSGGSAKNTITKTLKLRIVRPYNSAEVEKIVADEKDNRERIALEKNKGKVKEACSKHLKVAAYCTTQVERNACLFCKARKLDDKFYQELRGQFPDAVFWQEIGEIFRQLQKQAAEIYNQSLIELYYEIFIKGKGIANASSVGHYLSDVCYTRAAELFKNAAIASGLRSKIKSNFRLKELRNMRGGLPTTKSDNFPIPLVKQKGGQYTGFEISSHNDDFIIKIPFGRWQVKKEIDKYRPWEKLDFEQVRKSPKPISLLLSTQRRKRNKGWSKDEGTEAEIRKVMNGDYQTSYIEVKRGSKIGEKSTWMLNLSIDVPKIDKGVDPSIVGGIDVGVKSPLVCAIDNVLSRYSISDNDLFHFNKKMFARRRILLKKNRHRRAGHGAKNKLRPISILTERSGRFRKKLIERWACEIADFFIRNKVGTVQMENLESMKRREDSYFNIRLRGFWPYAEMQNKIEFKLKQYGIEIRKVAPNNTSKTCSKCGHLNNYFNFEYRKKNKFPYFKCEKCNFKENADYNAALNISNPKLKSTKEEP

SEQ ID NO: 2489 - protein, 726 aa, synthetic construct
SEVEFSHEYWMRHALTLAERARDEREVPVGAVLVLNNRVIGEGWNRAIGLHDPTAHAEIMALRQGGLVMQNYRLVDATLYVTFEPCVLCAGAMVHSRIGRVVFGVRNSKRGAAGSLMNVLNYPGMNHRVEITEGILADECAALLCDFYRMPRQVFNARKKARSNINSGGSSGGSSGSETPGTNGSATPESSGGGSGGSAKNTITKTLKLRIVRPYNSAEVEKIVADEKNNREKIALEKNKDKVKEACSEHLKVAAYCTTQVERSACLFCKARKLDDKFYQKLRGQFPDAVFWQEISEIFRQLQKQAAEIYNQSLIELYYEIFIKGKGFANASSVEHYLSDVCYTRAAELFKNAAIASGLRGKVKSNFRLKVLKSMKGGLPTTKSDNFPIPLVKQKGGQYTGFEISSHNDDFIIKIPFGRWQVKKEIDKYRPWEKFDFEQVRKSPKPISLLLSTQRRKRNKGWSKDEGTEAEIRKVMNGDYQTSYIEVKRGSKTGEKSAWMLNLSIDVPKIDKGVDPSIIGGIDVGVKSPLVCAINNAFSRYSISDNDLFHFNKKMFARRRILLKKNGHKRAGHGARNKLKPITVLTEKSKRFRKKLIERWACEIANFFIKNRVGTVQMENLESMKRKEDSYFNIRLRGFWPYAEMQNRIEFKLEQYGIKIRKVAPNNTSKTCSKCGHLNNYFNFEYRKKNKFPHFKCEKCNFKEDADYNAALNISNPKLKSTKEEP

SEQ ID NO: 2490 - protein, 726 aa, synthetic construct
SEVEFSHEYWMRHALTLAKRARDEREVPVGAILVLNNRVIGVGWNRAIGLHDPTAHAEIMALRQGGLVMQNYRLIDATLYVTFEPCVMCAGAMIHSRIGRVVFGVRNSKHGAAGSLVNVLNYPGMNHRVEITEGILADECAALLCDFYRMPRQVFNARKEAQSSINSGGSSGGSSGSETPSTSESTTPESSGGSSGGPAKNTITKTLKLRIVRPYNSAEVEKIVADEKNNREKTALEKNKDKVKEACSKHLKVAAYCTTQVERNACLFCKARKLDDKFYQKLRGQFPDAVFWQELGEILRQLQKQAAEIYNQSLIELYYEIFIKGRGFANASSVEHYLSDVCYTRAAELFKNAAIASGLRGKVKSNFRLKELKNMKSGLPTTKSDNFPIPLVKQKGGQYTGFEISSHNDDFIIKIPFGRWQVKKEIDKYRPWEKFDFEQVRKSPKPISLLLSTQRRKRNKGWSKDEGTEAEIRKVMNGDYQTSYIEVKRGSKIGEKSAWMLNLSIDVPKIDKGVDPSIIGGVDVGVKSPLVCAINNALSRYSISDNDLFRFNKRMFARRRILLKKNRHKRAGHGAKNKLKPVSILTEKSERFRKKLIERWACEIADFFIKNKVGTVQMENLESMKRKEDSYFNIRLRGFWPYAEMQNKIEFKLKQYGIEIRKVAPNNTSKTCSKCGHLNNYFNFEYRRKNKFPHFKCEKCNFKENADYNAALNISNPKLKSTKEEP

SEQ ID NO: 2491 - protein, 726 aa, synthetic construct
SEVEFSHEYWMRHALSLAKRARDEREVPVGAVLVLNNRIIGEGWNRAIGLHDPTAHAEIMALRQGGLVMQNYRLIDATLYVTFEPCVMCAGAMIHSRIGRVVFGVRNSKHGAAGSLVNVLNYPGMNHRVGITEGILADECAALLCDFYRMPRQVFNARKKAQSSINPGGSSGGSSGSETQGTSESATPESSGGSSGGSAKNTITKTLKLRIVRPYNSAEVEKVVADEKNNREKIALEKNKDKVKEACSKHLKVASYCTTQVERNACLFCKARKLDDKFYQKLRGQFPDAVFWQELGEIFRQLQKQAAEVYNQSLIELYYEIFIKGKGFANASNVEHYLSDVCYTRAAELFKNAAIASGLRSKIKSNFRLKELRNMKSGLPTTKSDNFPIPLVKQKGGQCTGFEISNHNSDFIIKIPFGRWQVKKEIDKYRPWEKFDFEQVRKSPKPISLLLSTQRRRRNKGWSKDEGTEAEIRKVMNGDYQASYIEVKRGSRIGEKSAWMLNLSIDVPKIDKGVDPSIIGGIDVGVKSPLVCAINNAFSRYSISDNDLFHFNKKVFARRRILLKKNRHRRAGHGTKNKLKPITILTEKSKRFRKKLIERWACEIADFFIKNKVGTVQMENLESMKRKEDSYFNIRLRGFWPYAEMQNKIEFKLKQYGIEIRKVAPNNTSKTCSKCGHLNNYFNFEYRKKNKFPHFKCEKCNFKENADYNAALNISNPKLKSTKEKP

SEQ ID NO: 2492 - protein, 726 aa, synthetic construct
SEVEFSHEYWMRHALTLAERARDAREVPVGAILVLNNRVIGEGWNRAIGQHDPTAHAEIMALRQGGLVMQNYRLIDATLYVTFEPCVMCAGAMIHSRIGRVVFGVRNSKHGAAGSLMNVLNYPGMNHRVEITEGILADECAALLCDFYRMPRQVFNGRKKAQSSINSGGPSGGSSGSETPSTSESATPESSGGSSGGSAKNTITKTLTLRIVRPYNSAEVEKIVADEKNNREKIALEKNKDKVKEACSEHLKVAAYCTTQVERSACLFCKARKLDDKFYQKLRGQFPDAVFWQEIGEIFRQLQKQAAEVYNQSLIELYYEIFIKGKGFANASSVEHYLSDVCYTRAAELFKNAAIASGLRGKVKSNFRLKELRNMKSGLPTTKSDNFPIPLVKQKGGQYTGFEISSHNDDFIIKIPFGRWQVKKEIDKYRPWEKFDFEQVRKSPKPISLLLSTQRRKRNKGWGKDEGTEAEIRKVMNGDYQTSYIEVKRGSKIGEKSAWMLNLSIDVPKLDKGVDPSIIGGIDVGVKSPLVCAINNAFSRYSISDNDLFHFNKKMFARRRILLKKNRHRRAGHGAKNKLKPISILTEKSKRFRKKLIERWACEIADFFIKNKVGTVQMENLESMKRKEDSYFNIRLRGFWPYAEMQNKIEFKLKQYGIEIRKVAPNNTSKTCSKCGHLNNYFNFEYRRKNKFPHFKCEKCNFKENADYNAALNISNPKLKSTKEEP

SEQ ID NO: 2493 - protein, 726 aa, synthetic construct
SEVEFSHEYWMRHALTLAKRARDEREVPVGAILVLNNRVIGEGWNRAIGLHDPTAHAEIMALRQGGLVMQNYRLIDATLYVTFEPCVMCAGAMIHSRIGRVVFGVRNNKHGAAGSLVNVLNYPGMNHRVEITEGVLADECAALLCDFYCMPRQVFNAQKRAQSSINSGGSSGGSSGSVTPGTSESATPESSGGGSSGSAKNTITKTLQLRIVRPYNSAEVEKIVADEKNNREKIALEKNKDKVKEACSKHLKVASYCTTQVERNACPFCKARKLDDKFYQKLRGQFPDAVFWQELGEILRQLQKQAAEVYNQSLIELYYEIFIKGKGFANASNVEHYLSDVCYTRAAELFKNAAIASGLRGKVKSNFRLKELKNMKSGLPTTKSDNFPIPLVKQKGGQYTGFEIRSHSDDFIIKIPFGRWQVRKEIDKYRPWEKFDFEQVRKSPKPISLLLSTQRRKRNKGWSKDEGTEAEIRKVMNGDYQTSYIEVKRGSKAGEKSAWMLNLSIDVPKIDKGVDPSIIGGIDVGVKSPLVCAINNALSRYSISDNDLFHFNKKMFARRRILLRKNRHKRAGHGAKNKLKPITMMTEKSKRFRKKLIERWACEIADFFIKNKVGTVQMENLESMKRKEDSYFNIRLRGFWPYAEMQNKIEFKLKQYGIEIRKVAPNSTSKTCSKCGHLNNYFNFEYRKRNKFPHFKCEKCNFKENADYNAALNISNPKLKGTKEEP

SEQ ID NO: 2494 - protein, 726 aa, synthetic construct
SEVEFSHEYWMRHALTLAKRARDEREVPVGAILVLNNRVIGEGWNRAIGLHDPTAHAEIMALRQGGLVMQNYRLIDATLYVTFEPCVMCAGAMIHSRIGRVVFGVRNNKHGAAGSLVNVLNYPGMNHRVEITEGILADECAALLCDFYRMPRQVFNARKKAQSSINPGGSSGGSSGSETPGTSESATPESSGGSSSGSAKNTITKTLQLRIVRPYNSAEVEKIVADEKNNREKIALEKNKDKVKEACSKHLKVASYCTTQVERNACPFCKARKLDDKFYQKLRGQFPDAVFWQELGEIFRQLQKQAAEIYNQSLIELYYEILIKGKGFANACSVEHYLSDVCYTRAAELFKNAAIASGLRSKIKSNFRLKELKNMKSGLPTTKSDNFPIPLVKQKGGQYTGFEISNHNGDFIIKIPFGGWQVKKEIDKYRPWEKFDFEQVRKSPKPISLLLSTQRRKRNKGWSKDEGTEAEIRKVMNGDYQTSYIEVKRGSKTGEKSAWMVNLSIDVPKIDKGVDPSIIGGIDVGVKSPLVCAVNDALSRYSINDNDLFHFNKKMFARRRILLKKNGHKRAGHGAKNKLKPITTLTEKSKRFRKKLIERWACEIADFFIKNKVGTVQMENLESMKRKEDSYFNIRLRGFWPYAEMQNKIEFKLRQYGIEIRKVAPNNTSKTCSKCGHLNNYFDFEYRKKNKFPHFKCEKCYFKEDADYNAALNISNPRLKSTKEEP

SEQ ID NO: 2495 - protein, 726 aa, synthetic construct
SEVEFSHEYWMRHALTLAKRARDEREVPVGAVLVLNNRVIGGGWNRAIGLHDPTAHAEIMALRQGGLVMQNYRLFDATLYVTFEPCVMCAGAMIHSRIGRVVFGVRNSKHGAAGSLVNVLNYPGMNHRVEITEGILADECAALLCDFYRMPRQVFNAQKKAQSSINPGGSSGGSSGSETRGTSESATPESSGGSSGGSAKNTITKTLKLRIVRPYNSAEVEKVVADEKNNREKIALEKNKDKVKEACSKHLKVASYCTTQVERNACLFCKARKLDDKFYQKLRGQFPDAVFWQELGEIFRQLQKQAAEIYNQSLIELYYEIFIKGKGITNASRVEHYLSDVCYTRAAELFKNAAIASGLRSKVRSNFRLKELKNMKSGLPTTKSDNFPIPLVKQKGGQYTGFEISSHNSDFIIKIPFGRWQEKEEIDKYRPWEKFDFEQVRKSPKPISLLLSTQRRKKNKGWSKDEGTEAEIRRVMNGDYQTSYIEVKRGSKIGEKSAWMLNLSIDVPKIDKGVDPSIIGGIDVGVKSPLVCAINNAFGRYSISDNDLFHFNKKMFARRRILLGKNRHKRAGHGAKNKLKPITILTEKSKRFRKKLIERWACEIADFFIKNKVGTVQMENLENMKRREDSYFNIRLRGFWPYAEMQNKIEFKLKQYGIEIRKVAPNNTSKTCSKCGHLNNYFNFEYRKRNKFPHFKCEKCNFKENADYNAALNISNPRLKSTKEEP

SEQ ID NO: 2496 - protein, 726 aa, synthetic construct
SEVEFSHEYWMRHALTLAKRARDEREVPVGAILVLNNRVIGEGWNRAIGLHDPTAHAEIMALRQGGLVMQNYRLIDATLYVTFEPCVMCAGAMIHSRIGRVVFGVRNNKHGAAGSLVNVLNYPGMNHRVEITEGILVDECAALLCDFYRMPRQVFNAQKKAQSTINSGGSSGGSSGSETPGTSESPTPESSGGSPGGSAKNTITKTLKLRIVRPYNSAEVEKIVVDEKNSREKIALEKNKDKVKEACSEHLKVAAYCTTQVERNACLFCKARKLDDRFYQKLRGQFPDAVFWQEVGEIFRQLQKQAAEIYNQSLIELYYEIFIKGKGFANASSVEHYLSDVCYTRAAELFKNAAIASGLRGKVKSNFRLKELKNMKSGLPTTKSDNFPIPLVKQKGGQYTGFEISSHNGDFIIKIPFGRWQVKKEIDKYRPWEKFDFEQVRKSPKPISLLLSTQRRKRNKGWSKDEGTEAEIRKVMNGVYQTSYIEVKRGSKIGEKSAWMLNLSIDVPKIDKGVDPSIIGGIDVGVKSPLVCAINNAFSRYGISDNDLFHFNKKMFARRRILLKKNRHKRAGHGAKNKLKPVSTLTEKSVRFRKKLIERWACEIADFFIKNKVGTVQMENLESMKRKEDSYFNIRLRGFWPYAEMQNKIEFKLKQYGIEIRKVAPNNTSKTCSKCGHLNNYFNFEYRKKNKFPHFKCEKCNFKENADYNAALNISNPKLKSTKEEP

SEQ ID NO: 2497 - protein, 726 aa, synthetic construct
SEVEFSHEYWMRHALTLAKRARDEREVPVGAILVLNNRVIGEGWNRAIGLHDPTAHAEIMALRQGGLVMQNYRLIDATLYVTFEPCVMCAGAMIHSRIGRVVFGVRNNKHGAAGSLVNVLNYPGMNHRVEITEGILVDECAALLCDFYRMPRQVFNAQKKAQSSINSGGSSGGNSGSETPSTSESATPESSGGSSGGSAKNTITKTLQLRIVRPYNSAEVEKIVTDEKNNREKIALEKNKDKVKEACSKHLKMAAYCTTQVERNACLFCKARKLDDKFYQKLRGQFPDAVFWQEIGEIFRQLQKQAAEIYNQSLIELYYEILIKGKGFANASSVEHYLSDVCYTRAAELFKNAAIASGLRGKVKSNFRLKELKNMKSGLPTTKSDNFPIPLVKQKGGQYTGFEISSHHDDFIIKIPFGRWQVKKEIDKYRPWEKFDFEQVRKSPKPISLLLSTQRRKRNKGWSKDEGTEAEIRKVMNGDYQISYIEVKRGSKIGEKSAWMLNLSVDVPKIDKGVDPSIVGGIDVGVKSPLVCAINNALSRYSISDNDLFHFNKKMFARRRILLRKNRYKRAGHGAKNKLKPISILTGKSERFRKKLIERWACEIADFFIKNKVGTVQMENLESMKRKEDSYFNIRLRGFWPYAEMQNRIEFKLKQYGIEIRKVAPNNTSKTCSKCGHLNNYFNFEYRRKNKFPHFKCEKCNFKENADYNAALNISNPKLKSTKEEP

SEQ ID NO: 2498 - protein, 726 aa, synthetic construct
SEVEFSHEYWMRHALTLAKRARDEREVPVGAVLVLNNRVIGEGWNRAIGLHDPTAHAEIMALRQGGLVMQNYRLIDATLYVTFEPCVMCAGAMIHSRIGRVVFGVRNNKHGAAGSLVNVLNYPGMGHRVEITEGILADECAALLCDFYCMPRQVFGARRKAQSSINPGGSSGGSSSSETPGTSESPTPESPGGSSGGSAKNTITKTLKLRIVRPYNSAEVEKIVADEKNNREKIALEKNKDKVKEACSKHLKVAAYCTTQVERNACLFCKARKLDDKFYQKLRGQFPDAVFWQEIGEIFRQLQKQAAEIYNQSLIELYYEIFIKGKGFANASSVEHYLSDVCYTRAAELFKNAAIASGLRGKVKSNFRLRELKNMKSGLPTTKSDNFPIPLVKQKGGQYTGFEISSHNDDFIIKIPFGRWQVKEEIDKYRPWEKFDFEQVRKSPKPISLLLSTQRRQKNKGWSKDEGTEAEIRRVMNGDYQTSYIEVKRGSKIGEKSTWMLNLSIDVPKIDKGVDPSIVGGIDVGVKSPLVCAINNSFSRYSICDNDLFRFNKKMFARRRILLKKNRHKRAGHGAKNKLKPITILTKKSERFRKKLIERWVCEVADFFIKNKVGTVQMENLESMKRKEDSYFNIRLRGFWPYAEMQNRIELKLKQYGIEIRRVAPNNTSRTCSKCGHLNNYFNFEYRKKSKFPHFKCEKCNFREDADYNAALNISNPKLKSTKEEP

SEQ ID NO: 2499 - protein, 726 aa, synthetic construct
SEVEFSHEYWMRHALTLAKRARDEREVPVGAILVLNNRVIGEGWNRAIGLHDPTAHAEIMALRQGGLVMQNYRLIDATLYVTFEPCVMCAGAMIHSRIGRVVFGVRNNKHGAAGSLVNVLNYPGMNHRVEITEGILADECAALLCDFYRMPRQVFNARKKAQSNINSGGSSGGSSGSEAPGTSESPTPESSGGGFGGSAKNTITKTLQLRIVRPYNSAEVEKIVADEKNSREKIALEKNKDKVKEACSKHLKVASYCTTQVERNACLFCRARRLDDEFYQKLRGQFPDAVFWQEIGEIFRQLQKQAAEIYNQSLIELYYEIFIKGKGIANASRVEHYLSDVCYTRAAELFKNAAIASGLRGKVKSNFRLKELKNMKSGLPTTKSDNFPIPLVRQKGGQYTGFEISSHNDDFIIKIPFGRWQVKKEIDKYRPWEKFDFEQVRKNPKPISLLLSTRRRKRNKGWSKDEGTEAEIRKVMNGDYQTSYIEVKRGSKIGEKSAWMLSLSIDVPKIDKGVDPSIIGGIDVGVKSPLVCAINNAFSRYSISDNELFHFNKKMFARRRILLRKNRHKRAGHGAKNKLKPISILTEKSKRFRKKLIERWACEIADFFIKNKVGTVQMENLESMKRREDSYFNIRLRGFWPYAKMQNKIEFKLKQYGIEIRKVAPNNTSKTCSKCGHLNNYFDFEYRKKNKFPHFKCEKCNFKESADYNAALNISNPKLKSTKEEP

SEQ ID NO: 2500 - protein, 726 aa, synthetic construct
GEDEFSHEYWMRHALTLAKRARDGREVPVGAVLVLNNRVIGEGWNRAIGLHDPTAHAEIMALRQGGLVMQNYRLIDATLYVTFEPCVMCAGAMVHSRIGRVVFGVRNSKRGAAGSLMNVLNYPGMNHCVEITEGILMDECAALLCDFYRMPRQVLNAQKKAQSSISSGGPSGGSSCSETPGASESVTPKSSGGSSTGSTKNTITKTLKLRIVRPYNSAEVEKIVADEKNSREKIALEKNKDKVKEACSEHLKVAAYCTTQVERNACLFCKARKLDDKFYQKLRGQFPDAVFWQEIGEIFRQLQKQAAEIYNQSLIELYYEIFIKGKGFANASSVEHYLSDVCYTRAAELFKNAAIASGLRGKVKSNFRLKELKNMKSGLPTTKSDNFPIPLVKQKGGQYTGFEISSHNDDFIIKIPFGRWQVKKEIDKYRPWEKFDFEQVRKSPKPISLLLSIQRRKRSKGWSKDEGTEAEIRKVMNGDYQTSYIEVKRGSKIGEKSAWMLNLSIDVPKIDKGVDPSIIGGIDVGVKSPLVCAVNNAFSRYSISDNELFHFNKKMFARRRILLKKNRHKRAGHGAKNKLKPISTLTERSKRFRKKLIERWACEIADFFIKNKVGTVQMENLESMKRKEDSYFNIRLRGFWPYAEMQNKIEFKLKQYGIEIRKVAPNNTSKTCSKCGHLNNYFNFEYRKKNKFPHFKCEKCNFKENADYNAALNISNPKLKSTKEEP

SEQ ID NO: 2501 - protein, 726 aa, synthetic construct
SEVEFSHEYWMRHALTLAKRARDEREVPVGAILVLNNRVIGEGWNRAIGLHDPTAHAEIMALRQGGLVMQNYRLIDATLYVTFEPCVMCAGAMIHSRIGRVVFGVRNNKHGAAGSLVNVLNYPGMNHRVEITEGILADDCAALLCDFYRMPRRVFNARKKAQSSTNPGGSFGGGSGSETPGTSESATLESSGGSSGGSAKNTITKTLKLRIVRPYNSAVVEKIVADEKNSREKIALEKNKDKVKEACSKHLKVASYCTTQVERNACLFCKARKLDDKFYQKLRGQFPDAVFWQELGEIFRQLQKQAAEIYNQSLIELYYEIIIKGKGFANASSVEHYLSDVCYTRAAELFKNAAIASGLRGKVKSNFRLKELKNMKSGLPTTKSDNFPIPLVKQKGGQYTGFEISSHNDDFIIKIPFGRWQVKKEIDKYRPWEKFDFEQVRKSPKPISLLLSTQRRKRSKGWSKDEGTEAEIRKVMNGDYQTSYIEVKRGSKIGEKNAWMLNLSIDVPKIDKGVDPSIIGGIDVGVKSPLVCAINNALGRYSISDNDLFHFNKKMFARRRILLKKNRHKRAGHGVRNKLKPITVLTEKSERFRKKLIERWACEIANFFIKNKVGTVQMENLEGMKRREDSYFNIRLRGFWPYAEMQDKIEFKLKQYGIEIRKVAPNNTSKTCSRCGHLNNYFNFEYRRKNKFPHFKCEKCNFKENADYNAALNISNPKLKSSKEEP

SEQ ID NO: 2502 - protein, 726 aa, synthetic construct
SEVEFSHEYWMRHALTLAKRARDEREVPVGAILVLNNRVIGEGWNRAIGLHDPTAHAEIMALRQGGLVMQNYRLIDATLYVTFEPCVMCAGAMIHSRIGRVVFGVRNSKHGAAGSLVNVLNYPGMNHCVEITEGILVDECAALLCDFYRMPRQVLNAQKKAQSSISPGGSSGGSSGSETPGASGSVTPKSSGGSSAGSTKDTITKTLKLRIVRPYNSAEVEKIVADEKNSREKIALEKYKDKVKEACSEHLKVAAYCTTQVERNACLFCKARKLDDRFYQKLRGQFPGAVFWQEIGEIFRQLQKQAAEIYNQSLIELYYEIFIKGKGFANASSVEHYLSDVCYTRAAELFKNAAIASGLRGKVKSNFRLKELKNMKSGLPTTKSDNFPIPLVKQKGGQYTGFEISNHNGDFIIKIPFGRWQVKKEINRYRPWEKFDFEQVRKSPKPISLLLSTQRRKRNKGWSRDEGTEAEIRKVMNGDYQTSYIEVKRGSKIGEKSAWMLNLSIDVPKIDKGVDPSIIGGIDVGVKSPLICAINNAFSRYGISDNDLFRFNKKVFARRRILLKKNRHKRAGHGTKNKLKPITILTEKSGRFRKKLIERWACEIANFFIKNKVGTVQMENLDSMKRKEDSYFNIRLRGFWPYAEMQNKIEFKLKQYGIKIRKVAPNNTSKTCSKCGHLNNYFSFEYRKKNKFPHFKCEKCNFKEDADYNAALNISNPKLKSTREEP

SEQ ID NO: 2503 - protein, 726 aa, synthetic construct
SEVEFSHEYWMRHALTLAKRARDEREVPVGAVLVLNNRVIGEGWNRAIGLHDPTAHAEIMALRQGGLVMQNYRLVDATLYVTFEPCVLCAGAMVHSRIGRVVFGARNSKRGAAGSLMNVLNYPGMNHRVEITEGILADECAALLCDFYRMPRQVFNARKKARSNINSSGSSGGSSGSETPGTSESATPESSGGSSGGSAKNTITKTLKLRIVRPYNSAEVEKIVADEKNNREKIALETNKDKVKEACSKHLKVASYCTTQVERNACLFCKARKLDDKFYQKLRGQFPDAVFWQELGEIFRQLQKQAAEIYNQSLIELYYEIFIKGKGITNASRVEHYLSDVCYTRAAELFKNAAIASGLRSKVRSNFRLKELKNMKSGLPTTKSDNFPIPLVKQKGGQYTGFEISSHNSDFIIKIPFGRWQEKEEIDKYRPWEKFDFEQVRKSPKPISLLLSTQRRKKNKGWSKDEGTEAEIRRVMNGDYQTSYIEVKRGSKIGEKSAWMLNLSIDVPKIDKGVDPSIIGGIDVGVKSPLVCAINNAFSRYSISDNDLFHFNKKMFARRRILLKKNRHRRAGHGAKNKLKPITILTEKSVRFRKKLIERWACEIADFFIKNKVGTVQMENLESMKRKEDSYFNIRLRGFWPYAEMQNKIEFKLKQYGVEIRRVAPNNTSRTCSKCGHLNNYFNFEYRRKNKFPHFKCEKCNFKEDADYNAALNISNPKLKSTKEEP

SEQ ID NO: 2504 - protein, 726 aa, synthetic construct
SEVEFSHEYWMRHALTLAERARDEHEVPVGAVLVLNNRVIGEGWNRAIGLHDPTAHAEIMALRQGGLVMQNYRLIDATLYVTFEPCVMCAGAMIHSRIGRVVFGVRNNKRGAAGSLMNILNYPGMNHRVEITEGILAGECAALLCDFYRMPRQALNAQKKAQSNTNSGGSSGGSSGSETPGTSESPTPESSGGSSGGSAKSTITKTLRLRIVRPYNSAEVEKIVADEKNNREKIALEKNKDKVKEACSKHLKVAAYCTTQVERNACLFCKARKLDDKFYQKLRGQFPDAVFWQELGGIFRQLQKQAAEIYNRSLIELYYEIFIKGKGITNASRVEHYLSDVCYTRAAELFKNAAIASGLRSKVRSNFRLKELKNMKSGLPTTKSDNFPIPLVKQKGGQYTGFEISSHNDDFIIKIPFGRWQVKKEIDRYRPWEKFDFEQVRKSPKPISLLLSTQRRKRNKGWSKDEGTEAEIRKAMNGDYQTSYIEVKRGSKIGEKSAWMLSLSIDVPKIDKGVDPRIIGGIDVGVKSPLVCAINNVLSRYSICDNDLFHFNKKMFARRRILLKKNRHRRAGHGARNKLKPITVLTEKSKRFRMKLIERWACEIANFFIKNKVGTVQMENLESMKRKEESYFNIRLRGFWPYAEMQNKIEFKLKQYGIEIRKVAPNNTSKTCSKCGHLNNYFNFEYRKKNKFPHFKCEKCNFKENADYNAALNISNPKLKSTKGEP

SEQ ID NO: 2505 - protein, 726 aa, synthetic construct
SEVEFSHEYWMRHALTLARRARDEREVPVGAILVLNNRVIGEGWNRAIGLHDPTAHAEIMALRQGGLVMQSYRLADATLYVTFEPCVMCAGAMIHSRIGRVVFGVRNSKHGAAGSLMNVLNYPGMNHRVEITEGILADECAALLCDFYRMPRQVFNARKKAQSSINSGGSSDGGSSSETPGTSESATPESSGGSSGGSAKNTITKTLKLRIVRPYNSAEVEKIVADEKNNREKIALEKNKDKVKEACSKHLKVAAYCTTQVERNACLFCKARRLDDKFYQKLRGQFPDAVFWQEIGEIFRQLQKQAAEIYNQSLVELYYEIFIKGKGIANASSVEHYLSDVCYTRAAELFKNAAIASGLRNKIKSNFRLKELRNMKSGLPTTKSDNFPIPLVRQKGGQYTGFEISSHNDDFIIKVPFGRWQVKKEIDKYRPWEKFDFEQVRKSPKPISLLLSTQRRKRNKGWSKDVGTEAEIRKVMNGDYQTSYIEVKRGSKIGEKSAWMLNLSIDVPKIDKGVDPSIIGGIDVGVRSPLVCAINNAFSRYSISDNDLFHFNKKMFARRRILLKKNRHKRAGHGAKNKLKPISILTEKSERFRKKLIERWACEIADFFIKNKVGTVQMENLESMKRREDSYFNIRLRGFWPYAKMQNKIEFKLKQYGIEIRKVAPNNTSKTCSKCGHLNNYFNFEYRKKNKFPHFKCEKCNFKESADYNAALNISNPKLKSTKEEP

SEQ ID NO: 2506 - protein, 726 aa, synthetic construct
SEVEFSHEYWMRHALTLAKRARDEREVPVGAVLVLNNRVIGEGWNRAIGLHDPTAHAEIMALRQGGLAMQNYRLVDATLYVTFEPCVLCAGAMVHSRIGRVVFGVRNSKRGAAGSLMNVLNHPGMNHRVEITGGILADECAALLCDFYRMPRQVFNAQKKARSNINSGGSSGGSSGSETLGTSESATPESSGGSPGGSAKNTITKTLKLRIVRPYNSAEVEKIVADEKNNREKIALEKNKDKVKEACSEHLKVAAYCTTQVERNACLFCKARKLDDKFYQKLRGQFPDAVFWQEISGIFRQLQKQAAEIYNQSLIELYYEIFIKGKGFANASSVEHYLSDVCYTRAAELFKNAAIASGLRGKVKSNFRLKELKSMKSGLPTTKSDNFPIPLVKQKGGQYTGFEISSHNDDFIIKVPFGRWQVKKEIDKYRPWEKFDFEQVRKSPKPISLLLSTQRRKRNKGWSKDVGTEAEIRKVMNGDYQTSYIEVKRGSKIGEKSAWMLNLSIDVPKIDKGVDPSIIGGIDVGVKSPLVCAINNAFSRYSISDNDLFHFNKKMFARRRILLKKNRHRRAGHGAKNKLKPIAVLTEKSEGFRKKLIERWACEVADFFIKNKVGTVQMENLESMKRREDSYFNIRLRGFWPYAEMQNKIEFKLRQYGIEIRKVAPNNTSKTCSKCGHLNNYFDFEYRKKNKFPHFKCEKCNFKENADYNAALNISNPKLRSTKEEP

SEQ ID NO: 2507 - protein, 726 aa, synthetic construct
SEVEFSHEYWMRHALTLAKRARDEREVPVGAILVLNNRVIGEGWNRAIGLHDPTAHAEIVALRQGGLAMQNYRLIDATLYVTFEPCVMCAGAMIHSRIGRVVFGVRNSKHGAAGSLVNVLNYPGMNHRVEITEGILADECAALLCDFYRMPRQVFGARRKAQSSINPGGSSGGSSSSETPGTSESPTPESPGGSSGGSAKNTITKTLKLRIVRPYNSAEVEKIVADEKNNREKIALEKNKDKVKEACSEHLKVAAYCTTQVERNACLFCKARKLDDKFYQKLRGQFPDAVFWQEISEIFRQLQKQAAEIYNQSLIELYYEIFIKGKGFANASSVEHYLSDVCYTRAAELFKNAAIASGLRGKVKSNFRLKELKNMKSGLPTTKSDNFPIPLVRQKGGQYTGFEISSHNDDFIIKIPFGRWQAKKEIDKYRPWEKFDFEQVRKSPKPISLLLSTQRRKRNKGWGKDEGTEAEIKKVMNGDYQTSYIEVRRGSKSGEKSAWMLSLSIDVPKIDKGVDPSIIGGIDVGVKSPLVCAINNAFSRYSISDNDLFRFNKKMFARRRILLKKNRHKRAGHGAKNKLKPITILTEKSVRFRKKLIERWACEIADFFIKNKVGTVQMENLESMKGKEDSYFNIRLRGFWPYAEMQNKIEFKLKQYGIEIRKVAPNNTSKTCSKCGHLNNYFNFEYRKKNKFPHFKCEKCYFKEDADYNAALNISNPRLKSTKEEP

SEQ ID NO: 2508 - protein, 726 aa, synthetic construct
SEVEFSHEYWMRHALTLAKRARDEREVPVGAVLVLNNRVIGEGWNRAIGLHDPTAHAEIMALRQGGLVMQNYRLIDATLYVTFEPCVMCAGAMVHSRIGRVVFGVRNSKHGAAGSLMNVLNYPGMNHRVEITEGILADECAGLLCDFYRMPRQVFSARKKAQSSINPGGSSGGSSGGEAPGTSESATLESSGGSSGDSAKNSITKTLQLRIVRPYNSAEVEKIVADEKDNREKTALEKNKDKVKEACSKHLKVASYCTTQVERNTCLFCKARKLDDKFYQKLRGQFPDAVFWQELGEIFRQLQKQAAEIYNQSLIELYYEIFIKGRGFANASSVEHYLSDVCYTRAAELFKNAAIASGLRGKVKSNFRLKELKNMKSGLPTTKSDNFPIPLVKQKGGQYTGFEISSHNDDFIIKIPFGRWQVKKEIDKYRPWEKFDFEQVRKSPKPISLLLSTQRRKRNKGWSKDEGTEAEIRKVMNGDYQTSYIEVKRGSKTGEKSAWMLNLSIDVPKIDKGVDPSIIGGIDVGVKSPLVCAINNAFSRYSISDNDLFRFNKKMFARRRILLKKNRHKRAGHGAKNKLKPISILTGKSERFRKKLIERWACEIADFFIKNKVGTVQMENLESMKRKEDSYFNIRLRGFWPYAEMQNKIEFKLKQYGIKIRKVAPNNTSKTCSKCGHLNNYFSFEYRKKNKFPHFKCEKCNFKEDADYNAALNISNPKLKSTKEEP

SEQ ID NO: 2509 - protein, 726 aa, synthetic construct
SEVEFSHEYWMRHALTLAKRARDEREVPVGAVLVLNNRVIGEGWNRTTGLHDPTAHAEIMALRQGGLVMQNYRLIDATLYVTFEPCVMCAGAMIHSRIGRVVFGVRNNKHGAAGSLVNVLNYPGMNHRVEITEGILADECAALLCDFYRMPRQVFNARKKAQSSINSGGSSGGNSGSETPGTSESATPGSSGGGSSGSAKNTITKTLQLRIVRPYNSAEVEKIVADEKNNRERVALEKNKDKVKEACSKHLKVAPYCTTQVERNACPFCKARKLDDKFYQKLRGQFPDAVFWQELGEILRQLQKQAAEIYNQSLIELYYEIFIKGRGFANASSVEHYLSDVCYTRAAELFKNAAIASGLRGKVKSNFRLKELKNMKSGLPTTKSDNFPIPLVKQKGGQYTGFEISSHNDDFIIKIPFGRWQVKKEINKYRPWEKFDFEQVRKSPKPISLLLSTQRRKRNKGWSKDEGTEAEIKKVMNGDYQISYIEVKRGSKIGEKSAWTLNLSVDVPKIDKGVDPSIIGGIDVGVKSPLVCAINNALSRYSISDNDLFHFNKKVFARRRILLKKNRHKRAGHGAKNKLKPISTLTERSKRFRKKLIERWACEIANFFVKNKVGTVQMENLESMKRKEDSYFNIRLRGFWPYAEMQNKIEFKLKQYGIKIRKVAPNNTSKTCSKCGHLNNYFSFEYRKKNKFPHFKCEKCNFKEDADYNAALNISNPKLKSTKEEP

SEQ ID NO: 2510 - protein, 726 aa, synthetic construct
SEVEFSHEYWMRHALTLAKRARDEREVPVGAVLVLNNRVIGEGWNRAIGLHDPTAHAEIMALRQGGLAMQNYRLVDATLYVTFEPCVLCAGAMVHSRIGRVVFGVRNSKRGAAGSLMNVLNHPGMNHRVEITEGILAGECAALLCDFYRMPRQVFNAQRKAQSNINPGGSSGGSSGSETPGTSESPTPESSGGSSGGSAKSTITKTLKLRIVRPYNSAEVEKIVADEKNNREKIALEKNKDKVRGACSRHLKVASYCTTQVERNACPFCKARKLDDKFYQKLRGQFPDAVFWQELGEIFRQLQKQAAEIYNQSLIELYYEIFIKGKGFANASSVEHYLSDVCYTRAAGLFKNAAIASGLRNKIKSNFRLKELKNMKSGLPTTRSDNFPIPLVKQKGGQYTGFEISSHNSDFIIKIPFGRWQVKEEIDKFRPWEKFDFEQVRKSPKPISLLLSTQRRKKNKGWSKDEGTEAEIRKVMNGDYQTSYIEVKRGSKIGEKGAWMLNLSIDVPKIDKGVDPSIIGGIDVGVKSPLVCAINNAFSRYSISDNDLFHFNKKMFARRRILLKKNRRRRAGHGAKNKLKPITILTRKSERFRKKLIERWACEIADFFIKNKVGTVQMENLESMKRKEDSYFNIRLRGFWPYAEMQNKIEFKLKQYGIEIRKVAPNNTSKTCSKCGHLNNYFNFEYRKKNKFPHFKCEKCNFKENADYNAALNISNPKLKSTKEKP

SEQ ID NO: 2511 - protein, 726 aa, synthetic construct
SEVEFSHEYWMRHALTLAKRARDEREVPVGAVLVLNNRVIGEGWNRAIGLHDPTAHAEIMALRQGGLVMQNYRLTDATLYVTFEPCVMCAGAMIHSRIGRVVFGVRNSKRGAAGSLMNVLNYPGMNHCVEITEGILVDECAALLCDFYRMPRQVLNAQKKAQSSISSGGSSGGSSCSETPGASESVTPKSSGGSSAGSTKNTITKTLKLRIVRPYNSAEVEKIVADEKNSREKIALEKNKDKVKEACSEHLKVAAYCTTQVERNACLFCKARKLDDRFYQELRGQFPDAVFWQEIGEIFRQLQKQAAEIYNQSLIELYYEIFIKGKGFANASSVEHYLSDVCYTRAAELFKNAAIASGLRGKVKSNFRLKELKNMKSGLPTTKSDNFPIPLVRQKGGQYTGFEISSHNSDFIIKIPFGRWQVKEEIDKFRPWEKFDFEQVRKSPKPISLLLSTQRRRRNKGWSKDEGTEAEIRKVMNGDYQTSYIEVKRGSKIGEKGAWMLNLSIDVPRIDKGVDPSIIGGIDVGVKSPLVCAINNAFSRYSISDNDLFHFNKKMFARRRILLKKNRHKRAGHGAKNKLKPISILTEKSKRFRKKLIERWACEIADFFIKNKVGTVQMENLESMKRKEDSYFNIRLRGFWPYAEMQNKIEFKLKQYGIEIRKVAPNNTSKTCSKCGHLNNYFNFEYRRKNKFPHFKCEKCNFKEDADYNAALNISNPELKSTKEEP

SEQ ID NO: 2512 - protein, 726 aa, synthetic construct
SEVEFSHEYWMRHALTLAKRARDEREVPVGAILVLNNRVIGEGWNRAIGLHDPTAHAEIMALRQGGLVMQNYRLTDATLYATFEPCVMCAGAMIHSRIGRVVFGVRNSKHGAAGSLMNVLNYPGMNHRVEITEGILADECAGLLCDFYRMPRQVFSARKKAQSSINPGGSSGGSSGGKAPGTSESATLESSGGSSGDSAKNSITKTLKLRIVRPYNSAEVEKIVADEKNSREKIALEKNKDKVKEACSKHLKVAAYCTTQVERNACPFCKARKLDDKFYQKLRGQFPDAVFWQELGEILRQLQKQAAEIYNQSLIELYYEIFIKGRGFANASSVEHYLSDVCYTRAAELFKNAAIASGLRGKVKSNFRLKELKNMKSGLPTTKSDNFPIPLVKQKGGQYTGFEISSHNDDFIIKIPFGRWQVKKEIDKYRPWEKFDFEQVRKSPKPISLLLSTQRRKRNKGWSKDEGTEAEIRKVMNGDYQTSYIEVKRGSKIGEKSAWMLNLSIDVPKIDKGVDPSIIGGIDVGVKSPLVCAINNAFSRYSISDNDLFRFNKKMFARRRILLKKNRHKRAGHGAKNKLKPISILTGKSERFRKKLIERWACEIADFFIKNKVGTVQMENLESMKRKEDSYFNIRLRGFWPYAEMQNKIEFKLKQYGIEIRKVAPNNTSKTCSKCGHLNNYFNFEYRRKYKFPHFKCEKCNFKEDADYNAALNISNPKLKSTKEEP

SEQ ID NO: 2513 - protein, 726 aa, synthetic construct
SEVEFSHEYWMRHALTLAKRARDEREVPVGAVLVLNNRVIGEGWNRAIGLHDPTAHAEIMALRQGGLVLQNYRLVDATLYVTFEPCIMCAGAMIHSRIGRVVFGVRNSKRGAAGSLMNVLDYPGMNHRVEITEGVLADECAALLCDFYRMPRQVLNAQKMAQSSINSGGSSGGSSGSKTPGTSESATPESSGGSSGGSAKNSITKTLKLRIVRPYNSAEVEKIVADEKNNREKIALEKNKGKVKEACSKHLKVATYCTTQVERNACLFCKARKLDDKFYQKLRGQFPDAVFWQEIGEIFRQLQKQAAEIYNQSLIELYYEIFIKGKGIANASSVEHYLSDVCYTRAAELFKNAAIASGLRNKIKSNFRLKELKNMKSGLPTTKSDNFPIPLVKQKGGQYTGFEISSHNDDFIIKIPFGRWQVRKEIDKYRPWEKFNFEQVRKSPKPISLLLSTQRRKRNKGWSKDEGTEAEIRKVMNGDYQTSYIEVKRGSKIGEKSAWMLSLSIDVPKIDKGVDPSIIGGIDVGVKSPLVCAINNAFNRYSISDNNLFHFNKKMFARRRILLKKNRHKRAGHGAKNKLKPISILTGKSERFRKKLIERWACEIADFFIKNKVGTVQMENLESMKRKEDSYFNIRLRGFWPYAEMQNKIEFKLKQYGIEIRKVAPNNTSKTCSKCGHLNNYFNFEYRKKNKFPHFKCEKCNFKESADYNAALNISNPKLKSTKEEP

SEQ ID NO: 2514 - protein, 726 aa, synthetic construct
SEVEFSHEYWMRHALTLAKRARDEREVPVGAVLVLNNRVIGEGWNRTTGLHDPTAHAEIMALRQGGLVMQNYRLTDATLYVTFEPCVMCAGAMIHSRIGRVVFGVRNSKRGAAGSLMNVLNYPGMNHCVEITEGILMDECAALLCDFYRMPRQVLSAQKKAQSSISSGGPSGGSSCSETPGASESVTPKSSGGSSGGSAKNTITKALKLRIVRPYNSAEVEKIVADEKNNRERIALEKNKDKVKEACSKHLKVAAYCTTQVERNACLFCKARKLDDKFYQKLRGQFPDAVFWQEIGEIFRQLQKQAAEIYNQSLIELYYEIFIKGKGFANASSVEHYLSGVCYTRAAELFKNAAIASGLRGKVKSNFRLKELKNMRSGLPTTKSDNFPIPLVKQKGGQYAGFEISSHNDDFIIKIPFGRWQVKKEIDKYRPWEKFDFEQVRKSPKPISLLLSTRRRKRNKGWSKDEGTEAEIRKVMNGDYQTSYIEVKRGSKIGEKSAWMLNLSIDVPKIDKGVDPSIIGGIDVGVKSPLVCAINNAFGRYSISDNDLFHFNKKMFARRRILLKRNRHRRAGHGAKNKLKPITILTEKSKRFRKKLIERWACEIADFFIKNKVGTVQMENLESMKRKEDSYFNIRLRGFWPYAEMQNKIEFKLKQYGIEIRKVAPDNTSKTCSKCGHLNNYFNFEYRRKNKFPHFKCEKCNFKEDADYNAALNISNPKLKSTKEEP

SEQ ID NO: 2515 - protein, 726 aa, synthetic construct
SEVEFSHEYWMRHALTLAKRARDEREVPVGAVLVLNNRVIGEGWNRTAGLHDPTAHAEIMALRQGGLVMQNHRLIDATLYVTFEPCVMCAGAMIHSRIGRVVFGVRNSKRGAAGSLMNVLNYPGMGHCVEITEGILADECAALLCDFYRMPRQVLNAQKKAQSSISSGGSSGGSSGSETPGASGSVTPKSSGGSSAGSTKDTITKTLKLRIVRPYNSAEVEKVVADEKNNREKIAIEKNKDMVKEACSKHLKVASYCTTQVERNACLFCKARKLDDKFYQKLRGQFPDAVFWQELGGIFRQLQKQAAEIYNQSLIELYYEIFIKGKGITNASRVEHYLSDVCYTRAAEQFKNAAIASGLRSKVRSNFRLKELKNMKSGLPTTKSDNFPIPLVKQKGGQYTGFEISSHNDDLIIKIPFGRWQVKREIDKYRPWEKFDFEQVRKSPKPISLLLSTQRRKRNKGWSKDEGTEAEIRKVMNGDYQTSYIEVKRGSKIGEKRAWMLNLSIDVPKVDKGVDPSIIGGVDVGVKSPLVCAINNAFSRYSISDNDLFRFNKRMFARRRILLKRNRHRRAGHGAKNKLKPISILTEKSERFRKKLIERWACEIADFFIKNKVGTVQMENLEGMKRKEDSYFNIRLRGFWPYAEMQNKIEFKLKQYGIEIRKVAPNNTSKTCSKCGHLNNYFNFEYRKKNKFPHFKCEKCNFKESADYNAALNISNPKLKSTKEEP

SEQ ID NO: 2516 - protein, 726 aa, synthetic construct
SEVEFSHEYWMRHALTLAKRARDEREVPVGAILVLNNRVIGEGWNRAIGLHDPTAHAEIMALRQGGLVMQNYRLIDATLYVTFEPCVMCAGAMIHSRIGRVVFGVRNSKHGAAGSLVNVLNYPGMNHRVEITEGILADECAALLCDFYRMPRQVFNARKKAQSSINPSGSSGGSSGSVTPGTSESATPESSGGSFGGSAKNTITKTLQLRIVRPYNSAEVEKIVADEKNSREKIALEKNKDKVKEACSKHLKVAAYCTTQVERNACLFCKARKLDDKFYQKLRGRFPDAVFWQELGEILRQLQKQAAEIYNQSLIELYYEIFIKGKGFANAGSVEHYLSDVCYTRAAELFKNAAIASGLRGKVKSNFRQKELKNMKSGLPTTKSDNFPIPLVKQKGGQYTGFEISSHNDDFIIKIPFGRWQVKKEIDKYRPWEKFDFEQVRKSPKPISLLLSTQRRKRNKGWSKDEGTEAEIRKVMNGDYQTSYIEVKRGSKTGEKSAWMLNLSIDVPKIDKGVDPSIIGGIDVGVKSPLVCAINNAFSRYSISDNDLFHFNKKMFARRRILLKKNGHKRAGHGAKNKLKPITILTEKSVRFRKKLIERWACEIADFFIRNKVGTVQMENLESMKRKEDSYFNIRLRGFWPYAEMQNKIEFKLKQYGIEIRKVAPNNTSKTCSKCGHLNNYFNFEYRKKNKFPHFKCEKCNFKENADYNAALNISNPKLRSTKEEP

SEQ ID NO: 2517 - protein, 726 aa, synthetic construct
SEVEFSHEYWMRHALTLAKRARDEREVPVGAILVLNNRVIGEGWNRAIGLHDPTAHAEIMALRQGGLVMQNYRLIDATLYVTFEPCVMCAGAMIHSRIGRVVFGVRNSKHGAAGSLMNVLNYPGMNHCVEITEGILVDECAALLCDFYRMPRQVLNAQKKAQSSISSGGSSGGSSGSETPGASGSVTPKSSGGSSAGSTKDTITKTLKLRIVRPYNSAEVEKIVADEKNSREKIALEKNKDKVKEACSKHLKVASYCTTQVERNACPFCKARKLDDKFYQKLRGQFPDAVFWQELGEILRQLQKQAAEIYNQSLIELYYEIFIKGRGFANASSVEHYLSDVCYTRAAELFKNAAIASGLRGKVKSNFRLKELKNMKSGLPTTKSDNFPIPLVKQKGGQYTGFEISSHNDDFIIKIPFGRWQVKKEIDKYRPWEKFDFEQVRKSPKPISLLLSTQRRKRNKGWSKDEGTEAEIRKVMNGDYQTSYIEVKRGSKTGEKSAWMLNLSIDVPKIDKGVDPSIIGGIDVGVKSPLVCAINNAFSRYSISDNDLFRFNKKMFARRRILLGKNRHKRAGHGAKNKLKPISILTGKSERFRKKLIERWACEIADFFIKNKVGTVQMENLESMKRKEDSYFNIRLRGFWPYAEMQNKIEFKLKQYGIEIRKVAPNNTSKTCSKCGHLNNYFNFEYRKKNKFPHFKCEKCNFKENADYNAALNISNPKLKSTKEEP

SEQ ID NO: 2518 - protein, 726 aa, synthetic construct; identical to SEQ ID NO: 684

SEQ ID NO: 2519 - protein, 726 aa, synthetic construct
SEVEFSHEYWMRHALTLAKRARDEREVPVGAVLVLNNRVIGEGWNRAIGLHDPTAHAEIMALRQGGLVMQNYRLIDATLYVTFEPCVMCAGAMIHSRIGRVVFGVRNNKHGAAGSLVNVLDYPGMNHRVEITEGILADECAALLCDFYRMPRQVFNARKKAQSSINPSGSSGGSSGSVTPGTSESATPESSGGGFGGSPKNTITKTLKLRIVRPYNSAEVEKIVADEKNNREKIALEKNKDKVKEACSKHLKVAAYCTTQVERNACLFCKARKLDDKFYQKLRGQFPDAVFWQELGEIFRQLQKQAAEIYNQSLIELYYVIFIKGKGLANASSVEHYLSDVCYTRAAELFKNAAIASGLRGKVKSNFKLKELKSMKSGLPSTKSDNFPIPLVKQRGGQYTGFEISSHNDDFIIKIPFGRWQAKKEIDKYRPWEKFDFEQVRKSPKPISLLLSTQRRKRNKGWSKDEGTEAEIKKVMNGDYQTSYIEVKRGSKIGEKSAWMLNLSIDVPKIDKGVDPSIIGGIDVGVKSPLVCAINNAFSRYSISDNDLFHFNKKMFARRRILLKKNRHRRAGHGAKNKLKPITILTEKSVRFRRKLIERWACEIADFFVKNKVGTVQMENLESMKRKEDSYFNIRLRGFWPYAEMQNKIEFKLKQYGIEIRKVAPNNTSKTCSKCGHLNNYFNFEYRRKNKFPHFKCEKCNFKEDADYNAALNISNPKLKSTKEEP

SEQ ID NO: 2520 - protein, 726 aa, synthetic construct
SEVEFSHEYWMRHALTLAKRARDEREVPVGAILVLNNRVIGEGWNRAIGLHDPTAHAEIMALRQGGLVMQNYRLIDATLYVTFEPCVMCAGAMIHSRIGRVVFGVRNSKHGAAGSLVNVLSYPGMNHRVEITEGILADECAALLCDFYRMPRQVLNAQKKAQSSISSGGSSGGSSGGKAPGTSESATLESSGGSSGGSAKNSITKTLKLRIVRPYNSAEVEKIVADEKNNREKIALEKNKDKVKEACSKHLKVASYCTTQVERNACLFCKARKLDDKFYQKLRGQFPDAVFWQELGEIFRQLQKQAAEIYNQSLIELYYEIFIKGKGFANASSVEHYLSDVCYTRAAELFKNAAIASGLRGKVKSNFRLKELKNMKSGLPTTKSDNFPIPLVKQKGGQYTGFEISSHNDDFIIKIPFGRWQVKKEINRYRPWEKFDFEQVRKSPKPISLLLSTQRRKRNKGWSKDEGTEAEIRKVMNGDYQTSYIEVKRGSKIGEKSAWMLNLGIDVPKIDKGVDPSIIGGIDVGVKSPLVCAINNAFSRFSISDNDLFHFNKKMFARRRILLKKNRHRRAGHGVKNKLKPITILAEKSKRFRKKLIERWACEIADFFVKNKVGTVQMENLESMKRKEDSYFNIRLRGFWPYAEMQNKIEFKLKQYGIEIRKVAPNNTSRTCSKCGHLNNYFNFEYRKKNKFPHFKCEKCNFKENADYNAALNISNPKLKSTKEEP

SEQ ID NO: 2521 - protein, 726 aa, synthetic construct; identical to SEQ ID NO: 684

SEQ ID NO: 2522 - protein, 726 aa, synthetic construct
SEVEFSHEYWMRHALTLAKRARDEREVPVGAVLVLNNRVIGEGWNRAIGLHDPTAHAEIMALRQGGLVMQNYRLTDATLYVTFEPCVMCAGAMIHSRIGRVVFGVRNSKRGAAGSLMNVLNYPGMNHCVEITEGILMDECAALLCDFYRMPRQVLSAQKKAQSSISSGGPSGGSSCSETPGTSESPTPESSGGSPGGSAKNTITKTLKLRIVRPYNSAEVEKIVADEKSNREKIALEKNKDKVKEACSKHLKVASYCTTQVERNACPFCKARKLDDKFYQKLRGQFPDAVFWQELGEILRQLQKQAAEIYNRSLIELYYEIFIKGRGFANASSVEHYLSDVCYTRAAELFKNAAIASGLRGKVKSNFRLKELKNMKSGLPTTKSDNFPIPLVKQKGGQYTGFEISSHNDDFIIKIPFGRWQVKKEIDKYRPWEKFDFEQVRKSPKPISLLLSTQRRKRNKGWSKDEGTEAEIRKVMNGDYQTSYIEVKRGSKAGEKSAWMLSLSVDVPKIDKGVDPSIIGGIDVGVKSPLVCAINNALSRYSISDNDLFHFNKKMFARRRILLRNNRHKRAGHGAKSKLKPITILTEKGERFRKKLIERWACEIANFFVKNKVGTVQMENLGSMKRKEDSYFNIRLRGFWPYAEMQNKIEFKLKQYGIEIRKVAPDNTSKTCSKCGHLNNYFNFEYRKKNKFPHFKCEKCNFKEDADYNAALNISNPKLKSTKEEP

SEQ ID NO: 2523 - protein, 726 aa, synthetic construct
SEVEFSHEYWMRHALTLAKRARDEREVPVGAILVLNNRVIGEGWNRAIGLHDPTAHAEIMALRQGGLVMQNYRLIDATLYVTFEPCVMCAGAMIHSRIGRVVFGVRNSKHGAAGSLVNVLNYPGMNHRVEITEGILADECAALLCDFYRMPRRVFSAQKKAQSTINSGGSSGGGSGSETPGTSESPTPESSGGSPGGSAKNTITKTLQLRIVRPYNSAEVEKIVTDEKNNRERIALEKNKDKVKEACSKHLKVASYCTTQVERNACPFCKARKLDDKFYQKLRGQFPDAVFWQELGEILRQLQKQAAEIYNQSLIELYYEIFIKGKGITNASRVEHYLSDVCYTRAAELFKNAAIASGLRSKVRSNFRLKELKSMKSGLPTTRSDNFPIPLVKQKGGQYTGFEISNHGSDFIIKIPFGRWQVKKEIDKYRPWEKFDFEQVRKSPKPISLLLSTQRRKRNKGWSKDEGTEAEIKKVMNGDYQISYIEVKRGSKIGEKSAWTLNLSIDVPKIDKGVDPSIIGGIDVGVKSPLVCAISNALSRYSINDNDLFHFNKKMFARRRILLKKSKHKRAGHGAKNKLKPITILTEKSRRFRKKLIERWACEIADFFIKNKVGTVQMENLEGMKRKEDSYFNIRLRGFWPYAEMQNKIEFKLKQYGIEIRKVAPNNTSKTCSKCGHLNNYFNFEYRKKNKFPHFKCEKCSFKENADYNAALNISNPKLKSTKEEP

SEQ ID NO: 2524 - protein, 726 aa, synthetic construct
SEVEFSHEYWMRHALTLARRARDEREVPVGAILVLNNRVIGEGWNRAIGQHDPTAHAEIMALRQGGLEMQNYRLIDATLYVTFEPCVMCAGAMIHSRIGRVVFGVRNSKHGAAGSLVNVLNYPGMNHRVEITEGILADECAALLCDFYRMPRQVFNARKKAQSSINPGGSSGGSSGSETPGTSESATPESSAGSSASSTKNTITKTLKLRIVRPYNSAEVEKIVADEKDNREKIALEKNKDKVKEACSKHLKVASYCTTQVERSACLFCKARKLDDKFYQKLRGQFPDAVFWQELGEIFRQLQKQAAEIYNQSLIELYYEIFIKGKGLANASSVEHYLSDVCYTRAAELFKNAAIASGLRGKVKSNFKLKELKNMKSGLPTTKSDNFPIPLVKQKGGQYTGFEISNHDGDFIIKIPFGRWQVKKEINKHRPWEKFDFEQVRKSPKPISLLLSTQRRKRNKGWSKDEGTEAEIRKVMNGDYQTSYIEVKRGSKIGEKSAWMLNLSIDVPKIDKGVDPSIIGGIDVGVKSPLVCAINNALSRYSISDNDLFHFNKKMFARRRILLRKNRHKRAGHGVRNKLKPITVLTEKSERFRKKLIERWACEIANFFIKNKVGTVQMENLESMKRREDSYFNIRLRGFWPYAEMQNKIEFKLKQYGIKVRKVAPNNTSKTCSKCGHLNNYFSFEYRKKNKFPHFKCEKCNFKENADYNAALNISNPKLKSTKEEP

SEQ ID NO: 2525 - protein, 726 aa, synthetic construct; identical to SEQ ID NO: 684

SEQ ID NO: 2526 - protein, 726 aa, synthetic construct
SEVEFSHEYWMRHALTLAKRARDEREVPVGAVLVLNNRVIGEGWNRAIGLHDPTAHAEIMALRQGGLVLQNYRLVDATLYVTFEPCVLCAGAMVHSRIGRVVFGARNSKRGAAGSLMNILNYPGMNHRVEITEGILADECAALLCDFYRMPRQVFNARKKAQSSINPGGSSGGSSGSETLGTSESATPESSGGSSGGSAKNTITKTLKLRIVRPYNSAEVEKIVADEKNSREKIALEKNKDKVKEACSKHLRVAAYCTTQVERNACLFCKARKLDDKFYQKLRGQFPDAVFWQELGEIFRQLQKQAAEIYNQSLIELYYEIFIKGKGIANASRVEHYLSDVCYTRAAELFKNAAIASGLRSKIKSNFRLKELRNMKSGLPTTMSDNFPIPLVKQKGGQYTGFEISNHNSDFIIKIPFGRWQVKEEIDKYRPWEKFDFEQVRKSPKPISLLLSTQRRKRSKGWSKDEGTEAEIRKVMNGDYQTSYIEVKRGSKIGEKSAWMLNLSIDVPKIDKGVDPSIIGGIDVGVKSPLVCAINNAFSRYSISDNDLFRFNKKMFARRRILLKKNRHKRAGHGAKNKLKPISILTKKSERFRKKLIERWVCEVADFFIKNKVGTVQMENLESMKRKEDSYFNIRLRGFWPYAEMQNRIELKLKQYGIEIRRVAPNNTSRTCSKCGHLNNYFNFEYRKKNKFPHFKCEKCNFREDADYNAALNISNPKLKSTKEEP

SEQ ID NO: 2527 - protein, 726 aa, synthetic construct; identical to SEQ ID NO: 684

SEQ ID NO: 2528 - protein, 726 aa, synthetic construct
SEVEFSHEYWMRHALTLAKRARDGREVPVGAVLVLNNRVIGEGWNRAIGLHDPTAHAEIMALRQGGLVMQNYRLIDATLYVTFEPCAMCAGAMVHSRIGRVVFGVRNSKRGAAGSLVNVLNYPGMNHRVEITEGILADECAALLCDFYRMPRQVFNARKKAQSSINPGGSSDGSSGSETPGTSESATPESPGGSSGGSAKNTITKTLKLRIVRPYNSAEVEKIVADEKNNREKSALEKNKDKVKEACSEHLKVAAYCTTQVERSACLFCKARKLDDKFYQKLRGQFPDAVFWQEIGEIFRQLQKQAAEIYNQSLIELYYEIFIKGKGFANASSVEHYLSDVCYTRAAELFKNAAIASGLRGKVKSNFRLKELKNMKSGLPTTKSDNFPIPLVKQKGGQYTGFEISSHNDDFIIKIPFGRWQVKKEIDKYRPWEKFDFEQVRKSPKPISLLLSTRRRKRNKGWSKDEGTEAEIRKVMNGDYQTSYIEVKRGSKIGEKSAWMLNLSIDVPKIDKGVDPSIIGGIDVGVKSPLVCAINNAPSRYSISDNDLFHFNKKMFARRRILLKKNRHKRAGHGVRNKLKPITALTEKSERFRKKLIERWACEIANFFIKNKVGTVQMENLESMKRKEDSYFNIRLRGFWPYAEMQNKIEFKLKQYGIEIRKVAPNNTSKTCSKCGHLNNYFNFEYRKKNKFPHFRCEKCNFRENADYNAALNISNPELKSTKEEP

SEQ ID NO: 2529 - protein, 726 aa, synthetic construct
SEVEFSHEYWMRHALTLAKRARDEREVPVGAVLVLNNRVIGEGWNRAIGLHDPTAHAEIMALRQGGLVMQNYRLADATLYVTFEPCVLCAGAMVHSRIGRVVFGVRNSKRGAAGSLMNVLNYPGMNHRVEITEGILADECAALLCDFYRMPRQVFNARKKARSNINSGGSSGGSSGSETPGTSESATPESSGGGSSGSAKNTITKTLQLRIVRPYNSAEVEKIVADEKNNREKIALEKNKDKVKEACSKHLKVASYCTTQVERSACPFCKARKLDDKFYQKLGGQFPDAVFWQELGEILRQLQKQAAEIYNQSLIELYYEIFIKGRGFANASSVEHYLSDVCYTRAAELFKNAAIASGLRGKVKSNFRLKELKNMKSGLPTTKSDNFPIPLVKQKGGQYTGFEISSHNDDFIIKIPFGRWQVKKEIDKYRPWEKFDFEQVRKSPKPISLLLSTQRRKRNKGWSKDEGTEAEIRKVMNGDYQTSYVEVKRGSKIGEKSAWMLNLSIDVPKIDKGVDPSIIGGIDVGVKSPLVCAVNNAFSRYSISDNDLFRFNKKMFARRRILLKKNRHQRAGHGAKNKLKPITILTEKSGRFRKKLIERWACEIADFFIKNKVGTVQMENLESMKRKEDSYFNIRLRGFWPYAEMQNKIVFKLKQYGIEIRRVAPNNTSRTCSKCGHLNNYFNFEYRRKYKFPHFKCEKCNFKEDADYNAALNISNPKLKSTKEEP

SEQ ID NO: 2530 - protein, 726 aa, synthetic construct
SEDEFSHEYWMRHALTLARRARDGREVPVGAVLVLNNRVIGEGWNRAIGLHDPTAHAEIMALRQGGLVMQNYRLIDATLYVTFEPCVMCAGAMVHSRIGRVVFGVRNSKRGAAGSLMNVLNYPGMNHCVEITEGILVDECAALLCDFYRMPRQVLNAQKKAQSSISSGGSSGGSSGSETPGASESVTPKSSGGSPGGSAKNTITKTLKLRIVRPYNSAEVEKIVADEKNNREKIALEKNKDKVKEACSKHLKVAAYCTTQVERNACLFCKARKLDDKFYQKLRGQFPDAVFWQEIGEILRQLQKQAAEIYNQSLIELYYEIFIKGKGFANASSVEHYLSDVCYTRAAELFKNAAIASGLRGKVKSNFRLKELKNMKSGLPTTKSDNFPIPLVKQKGGQYTGFEISSHNDDFIIKIPFGRWQVKEETDKYRPWEKFDFEQVRKNPKPISLLLSTQRRKRNKGWSKDEGTEAEIRKVMNGDYQTSYVEVKRGSKIGEKSAWMLNLSIDVPKIDKGVDPSIIGGIDVGVKSPLVCAVNNAFSRYSISDNDLFRFNKKMFARRRILLKKNRHQRAGHGAKNKLKPITILTEKSGRFRKKLIERWACEIADFFIKNKVGTVQMENLESMKRKEDSYFNIRLRGFWPYAEMQNKIVFKLKQYGIEIRRVAPNNTSRTCSKCGHLNNYFNFEYRRKYKFPHFKCEKCNFKEDADYNAALNISNPKLKSTKEEP

SEQ ID NO: 2531 - protein, 726 aa, synthetic construct
SEVEFSHEYWMRHALTLAKRARDEREVPVGAVLVLNNRVIGEGWNRAIGLHDPTAHAEIMALRQGGLVMQNYRLIDATLYVTFEPCVMCAGAMVHSRIGRVVFGVRNNKRGAAGSLMNVLDYPGMDHRVEITEGILADECAALLCDFYRMPRQVFNAQRKAQSSINSGGSSGGSSGSETPGTSESATPESSGGSSGGSAKNTITKTLQLRIVRPYNSAEVEKIVADEKNNREKIALEKNKDKVKEACSKHLKVASYCTTQVERNACPFCKARKLDDKFYQKLRGQFPDAVFWQELGEIFRQLQKQAAEIYNQSLIELYYEIFIKGKGFANASSVEHYLSDVCYTRAAELFKNAAIASGLRGKVKSNFRLKELKNMKGGLPTTKSDNFPIPLVKQKGGQYTGFEISSHNDDFIIKIPFGRWQAKKEIDKYRPWEKFDFEQVRKSPKPISLLLSTQRRKRNRGWSKDEGTEAEIRKVMNGDYQTSYIEVKRGSKIGEKSAWMLNLSIDVPKIDKGVDPSIIGGIDVGVKSPLVCAINNAFSRYSISDNDLFRFNKKMFARRRILLGKNRHKRAGHGVKNKLKPITILTEKSGRFRKKLIERWACEIADFFIKNRVGTVQMESLESMKRKEDSYFNIRLRGFWPYAEMQNKIEFKLKQYGIKIRKVAPNNTSKTCSMCGHLNNYFSFEYRKKNKFPHFKCEKCTFRENADYNAALNISNPKLRSTKEEP

SEQ ID NO: 2532 - protein, 726 aa, synthetic construct
SEVEFSHEYWMRHALALAKRARDEREVPVGAVLVLNNRVIGEGWNRAIGLHDPTAHAEIMALRQGGLVMQNYRLVDATLYVTFEPCVLCAGAMVHSRIGRVVFGVRNSKRGAAGSLMNVLNYPGMNHRVEITEGILADECAALLCDFYRMPRQVFNAQKKARSNINSGGSSGGSSGSETPGTSESATPESSGGSSGGSAKNTITKTLKLRIVRPYNSAEVEKIVADEKNNREKIALEKNKDKVKEACSKHLKVASYCTTQVERNACLFCKARKLDDRFYQRLRGQFPGAVFWQEIGEIFRQLQKQAAEIYNQSLIELYYEIFIKGKGIANASSVEHYLSDVCYTRAAELFKNAAIASGLRNKIKSNFRLKELRNMKSGLPTTKSDNFPIPLVRQKGGQYTGFEISNHNGDFIIKIPFGRWQVKEEINRHRPWEKFDFEQVRKSPKPISLLLSTQRRKRNKGWSRDEGTEAEIRKVMNGDYQTSYIEVKRGSKIGEKSAWMLNLSIDVPKIDKGVDPSIIGGIDVGVKSPLVCAINNALSRYSISDNDLFHFNKKMFARRRILLRKNRHKRAGHGARNKLKPITVLTEKSERFRKKLIERWACEIANFFIKNKVGTVQMENLESMKRREDSYFNIRLRGFWPYAEMQNKIEFKLKQYGIEIRKVAPNNTSKTCSKCGHLNNYFNFEFRKKNKFPRFKCEKCSFKEDADYNAALNISNPKLKSTKEEP

SEQ ID NO: 2533 - protein, 726 aa, synthetic construct
SEVEFSHEYWMRHALTLAKRARDEREVPVGAVLVLNNRVIGEGWNRTTGLHDPTAHAEIMALRQGGLVMRNYRLTDATLYVTFEPCVMCAGAMIHSRIGRVVFGVRNSKRGAAGSLMNVLNYPGMNHCVEITEGILVDECAALLCDFYRMPRQVLNAQKKAQSSVSSGGSSGGSSCSETPGASESVTPKSSGGGSAGSTKNTITKTLKLRIVRPYNSAEVEKIVADEKNSREKIALEKNKDKVKEACSEHLKVAAYCTTQVERNACLFCKARKLDDRFYQKLRGQFPDAVFWQEIGEVFRQLQKQAAEIYNQSLIELYYEIFIKGKGFANASSVEHYLSDVCYTRAAELFKNAAIASGLRGKVKSNFRLKELKNMKSGLPTTKSDNFPIPLVKQKGGQYTGFEISSHNDDFIIKIPFGRWQVKKEINKFRPWEKFDFEQVRKSPKPISLLLSTQRRKRNKGWSKDEGTEAEIRKVMNGDYQISYIEVKRGSRIGEKSAWMLSLSIDVPKIDRGVDPSIIGGIDVGVKSPLVCAINNALSRYSISDNDLFHFNKKVFARRRILLKKNRHRRAGHGAKNKLKPITILTEKSKRFRKKLIERWACEIANFFIKNKVGTVQMENLESMKGREDSYFNIRLRGFWPYAEMQSKIEFKLKQYGIKIRKVAPNNTSKTCSKCGHLNNYFNFEFRKKNKFPHFKCEKCNFKENADYNAALNISNPKLKSTKEEP

SEQ ID NO: 2534 - protein, 726 aa, synthetic construct
SEVEFSHEYWMRHALTLAKRARDEREVPVGAILVLNNRVIGEGWNRAIGLHDPTAHAEIMALRQGGLVMQNYRLSDATLYVTFEPCVMCAGAMIHSRIGRVVFGVRNSKRGAAGSLMNVLNYPGMNHCVEITEGILVDECAALLCDFYRMPRQVLSAQKKAQSSISSGGSSGGSSGSETPGTSGSVTPKSSVGSSAGSTKNTITKTLKLRIVRPYNSAEVEKIVADEKSNREKIALEKNKDKVKEACSKHLKVAAYCTTQVERNACLFCKARKLDDKFYQKLRGQFPDAVFWQEVGEIFRQLQKQAAEIYNQSLIELYYEIFIKGKGFANASSVEHYLSDVCYTRAAELFKNAAIASGLRGKVKSNFRLKELKNMKSGLPTTKSDNFPIPLVKQKGGQYTGFEISSHNDDFIIKIPFGRWQVKKEIDKYRPWEKFDFEQVRKSPKPISLLLSTQRRKRNKGWSKDEGTEAEIRKVMNGDYQTSYIEVKRGSKIGEKSAWMLNLSIDVPKIDKGVDPSIIGGIDVGVKSPLVCAINNAFSRYSISDNDLFRFNKKMFARRRILLKKNRHKRAGHGAKNKLKPISILTRKSERFRRKLIERWACEIADFFIKNKVGTVQMENLESMKRKEDSYFNIRLRGFWPYAEMQNRIELKLKQYGIEIRRVAPNNTSRTCSKCGHLNNYFNFEYRKKSKFPHFKCEKCNFREDADYNAALNISNPKLKSTKEGP

SEQ ID NO: 2535 - protein, 726 aa, synthetic construct; identical to SEQ ID NO: 684

SEQ ID NO: 2536 - protein, 726 aa, synthetic construct
SEVESSHEYWMRHALTLARRARDGREVPVGAVLVLNNRVIGEGWNRAIGLHDPTAHAEIMALRQGGLVMQNYRLIDATLYVTFEPCVMCAGAMVHSRIGRVVFGVRNSKRGAAGSLMNVLDYPGMGHRVEITEGILADECAALLCDFYCMPRQVFNAQKRAQSSINPSGSSGGSSGSVTPGTSESATPESSGGGFGGSAKNTITKTLQLRIVRPYNSAEVEKIVADEKNNREKIALEKNKDKVKEACSKHLKVASYCTTQVERNACLFCKARKLDDKFYQKLRGQFPDAVFWQELGEIFRQLQKQAAEIYNQSLIELYYEIFIKGRGFANAGSVEHYLSDVCYTRAAELFKNAAIASGLRGKVKSNFRLKELKNMKSGLPTTKSDNFPIPLVKQKGGQYTGFEISSHNSDFIIKIPFGRWQEKEEIDKYRPWEKFDFEQVRRSPKPISLLLSTQRRKRNKGWSKDEGTEAEIRKVMNGDYQTSYIEVKRGSKIGEKSAWMLNLSIDVPKIDKGVDPSIVGGIDVGVKSPLVCAIDNALSRYSISDNDLFHFNKKMFARRRILLKKNRHRRAGHGAKNKLKPISILTEKSKRFRKKLIERWACEIADFFIKNKVGTVQMENLESMKRKEDSYFNIRLRGFWPYAEMQNKIEFKLKQYGIEIRKVAPNNTSKTCSKCGHLNNYFNFEYRKMNKFPHFKCEKCNFKENADYNAALNISNPKLKSTKEEP

SEQ ID NO: 2537 - protein, 726 aa, synthetic construct
SEVEFSHEYWMRHALTLAKRARDEREVPVGAILVLNNRVIGEGWNRAIGLHDPTAHAEIMALRQGGLVMQNYRLIDATLYVTFEPCVMCAGAMIHSRIGRVVFGVRNNKHGAAGSLVNVLNYPGMNHRVEITEGILADECAALLCDFYRMPRQVFNARKKAQSSINPGGSSGGSSGGETPGTSESATPGSSGGSSGGSAKNTITKTLKLRIVRPYNSAEVEKIVADEKNNREKIALEKNKDKVKEACSKHLKVAAYCTTQVERNACLFCKARRLDDKFYQKLRGQFPDAVFWQEIGEIFRQLQKQAAEIYNQSLIELYYEIFIKGKGFANASSVEHYLSDVCYTRAAELFKNAAIASGLRGKVKSNFRLKELKNMKSGLPTTKSDNFPIPLVKQKGGQYTGFEISSHNDDFIIKIPFGRWQVKKEIDKYRPWEKFDFEQVRKSPKPISLLLSTQRRKRNKGWSRDEGTEAEIRKVMNGDYQTSYIEVKRGSKIGEKSAWMLSLSIDVPKIDKGVDPSIIGGIDVGVKSPLVCAINNAFSRYSISDNDLFRFNKKMFARRRILLGKNRHKRAGHGVKNKLKPITILTEKGGRFRKKLIERWACEIADFFIKNKVGAVQMENLESMKRKEDSYFNIRLRGFWPYAEMQDRIEFKLKQYGIEIRRVAPNNTSRTCSKCGHLNNYFNFEYRKKNKFPHFKCEKCNFREDADYNAALNISNPKLKSTKEEP

SEQ ID NO: 2538 - protein, 726 aa, synthetic construct
SEVEFSHEHWMRHALTLAKRARDEREVPVGAVLVLNNRVIGVGWNRAVGLHDPTAHAEIMALRQGGLVTQNYRLVDATLYVTFEPCVMCAGAMIHSRIGRVVFGVRNGKRGAAGSLMNVLNYPGMNHRVEITEGILADECAALLCDFYRMPCQVFNAQKKARSNINPGGSSGGSSGSETPGTSESPTPESSGGSSGGSAKSTITKTLKLRIVRPYNSAEVEKIVADEKNSREKIALEKNKDKVKEACSKHLKVAAYCTTQVERSACLFCKARKLDDKFYQKLRGQFPDAVFWQEIGEIFRQLQKQAAEIYNQSLIELYYEIFIKGKGFANASSVEHYLSDVCYTRAAGLFKNAAIASGLRGKVKSNFRLKELKNMKSGLPTTKSDNFPIPLVKQKGGQYTGFEISSHNDDFIIKIPFGRWQVKEEIDKYRPWEKFDFEQVRKNPKPISLLLSTQRRKRNKGWSKDEGTEAEIRKVMNGDYQTSYIEVKRGSKIGEKSAWMLNLSIDVPKIDKGVDPSIIGGIDVGVKSPLVCAINNAFSRYSISDNDLFRFNKKVFARRRILLKGNGHKRAGHGTKNKLKPITILTEKSERFRKKLIERWACEIADFFIKNKVGTVQMENLESMKRKEDSYFNIRLRGFWPYAEMQNKIEFKLRQYGIVVRKVAPNNTSKTCSKCGHLNNYFNFEYRKKNKFPHFKCEKCNFKEDADYNAALNVSNPKLKSTKEEP

SEQ ID NO: 2539 - protein, 726 aa, synthetic construct
SEVEFSHEYWMRHALTLARRARDEREVPVGAILVLNNRVIGEGWNRAIGLHDPTAHAEIMALRQGGLVMQSYRLADATLYVTFEPCVMCAGAMIHSRIGRVVFGVRNSKHGAAGSLMNVLNYPGMNHRVEITEGILVDECAALLCDFYRMPRQVLNAQKKAQSSVSSGGSSGGSSCSETPGASESVTPKSSGGGSAGSTKNTITKTLKLRIVRPYNSAEVEKIVADEKNSREKIALEKNKDKVKEACSEHLKVAAYCTTQVERNACLFCKARKLDDRFYQKLRGQFPDAVFWQEIGEIFRQLQKQAAEIYNQSLIELYYEIFIKGRGFANASSVEHYLSDVCYTRAAELFKNAAIASGLRGKVKSNFRLKELKSMKSGLPTTKSDNFPIPLVKQKGGQYTGFEISSHNDDFIIKIPFGRWQEKKEIDKYRPWEKFDFEQVRKSPKPISLLLSIQRRKRNKGWSKDEGTEAEIKKVMNGDYQTSYIEVKRGSRIGEKSAWMLSLSIDVPKIDRGVDPSIIGGIDVGVKSPLVCAINNAFSRYSISDNELFHFNKKMFARRRILLRKNRHKRAGHGARNKLKPITVLTEKSERFRKKLIERWACEIANFFVKNKVGTVQMEDLESMKRKEDSYFNIRLRGFWPYAEMQNKIEFKLKQYGIKIRKVAPNNTSKTCSKCGHLNNYFNFEYRKKNKFPHFKCEKCNFKEDADYNAALNISNPKLKSTKEEP

SEQ ID NO: 2540 - protein, 726 aa, synthetic construct
SEVEFSHEYWMRHALTLAKRARDEREVPVGAVLVLNNRVIGEGWNRAIGLHDPTAHAEIMALRQGGLVMQNYRLTDATLYVTFEPCVMCAGAMVHSRIGRVVFGVRNSKRGAAGSLMNVLNYPGMNHRVEVTEGILADECAALLCDFYRMPRQVFNAQKKARSNINSGGSSGGSSGSEMPGTSESATPESSGGNSGGSAKNTITKTLKLRIVRPYNSAEVEKIVADEKNNREKIALEKNKDKVKEACSEHLKVAAYCTTQVERNACLFCKARKLDDKFYQKLRGQFPDAVFWQEIGEIFRQLQKQAAEIYNQSLIELYYEILIKGKGFANASSVEHYLSDVCYTRAAELFKNAAIASGLRGKVKSNFRLKELKNMKSGLPTTKSDNFPIPLVKQKGGQYTGFEISSHNSDFIIKIPFGRWQAKKEIDRYRPWEKFDFEQVRKSPKPISLLLSTRRRKRNKGWSKDEGTEAEIRRVMNGDYQTSYIEVKRGSKIGEKSAWMLSLSIDVPKIDKGVDPRIIGGIDVGAKSPLVCAINNVLSRYSISDNDLFHFNKKMFARRRILLKKNGHKRAGHGAKNKLKPITIMTEKSKRFRKKLIERWACEIADFFIKNKVGTVQMENLESMKRKEDSYFNIRLRGFWPYAEMQNKIEFKLKQYGIEIRKVAPNNTSKTCSKCGHLNNYFNFEYRKKNKFPHFKCEKCNFKENADYNAALNISNPKLKSTKEEP

SEQ ID NO: 2541 - protein, 726 aa, synthetic construct
SEVEFSHEYWMRHALTLAKRARDECEVPVGAILVLNNRVIGEGWNRAIGLHDPTAHAEIMALRQGGLAMQNYRLIDATLYVTFEPCVMCAGAMIHSRIGRVVFGVRNNKHGAAGSLLNVLNYPGMNHRVEITEGILADECAALLCDFYRMPRQVFNARKKAQSSINPGGSSGGSSGSETPGTSESATPESSGGSSGGSAKNTITKTLKLRIVRPYNSAEVEKIVADEKNNREKIALEKNKDKVKVACSKHLKVASYCTTQVERNACPFCKARKLDDKFYQKLRGQFPDAVFWQELGGIFRQLQKQAAEIYNQSLIELYYEIFIKGKGITNASRVEHYLSDVCYTRAAELFKNAAIASGLRSKVRSNFRLKELRNMKSGLPTTKSDNFPIPLVRQKGGQYTGFEISNHNGDFIIKIPFGRWQVKKEINKHRPWEKFDFEQVRRSPKPISLLLSTQRRKKNKGWSKDEGTEAEIRRVMNGDYQTSYIEVKRGSKIGEKSAWMLNLSIDVPKIDKGVDPSIIGGIDVGVKSPLVCAINNSSSRYSISDNNLFHFNKKMFARRRILLKKNRHKRAGHGAKNKLKPISILTEKSERFRKKLIERWACEIADFFIRNKVGTVQMENLEGMKRREDSYFNIRLRGFWPYAEMQNKIEFKLKQYGIEVRRVAPNNTSKTCSKCGHLNNYFNFEYRKKNKFPHFKCEKCNFKENADYNAALNISNPKLKSTKEEP

SEQ ID NO: 2542 - protein, 726 aa, synthetic construct
SEVEFSHEYWMRHALTLAKRARDEREVPVGAVLVLNNRVIGVGWNRAIGLHDPTAHAEIMALRQGGLVMQNYRLIDATLYVTFEPCIMCAGAMIHSRIGRVVFGVRNSKRGAAGSLMNVLNYPGMNHRVEITEGVLADECAALLCDFYRMPRQVLNAQKKAQSSINSGGSSGGGSGSETPGTSESATQESSGGSSGGSAKNTITKTLKLRIVRPYNSAEVEKIVADEKNNREKIALEKNKDKVKEACSKHLKVASYCTTQVERNACLFCKARKLDDKFYQKLRGQFPDAVFWQELSEIFRQLQKQAAEIYNQSLIELYYEIFIKGKGFANASSVEHYLSDVCYTRAAELFKNAAIASGLRGKVKSNFRLKELKNMKSGLPTTKSDNFPIPLVKQKGGQYTGFEISSHNDDFIIKIPFGRWQVKREIDKYRPWEKFDFEQVRKSPKPISLLLSTQRRKRNKGWSKDEGTEAEIRKVMNGDYQTSYIEVKRGSKVGEKSAWMLNLSIDVPKIDKGVDPSIIGGIDVGVKSPLVCAVNNAFSRYSIGDNDLFHYNKKMFARRRILLKKNRHKRAGHGAKNKLKPITILTEKSVRFRKKLIERWACEIADFFVKNKVGTVQMENLESMKRKEDSYFNIRLRGFWPYAEMQNKIEFKLKQYGIEIRKVAPNNTSKTCSECGHLNNYFNFEYRKKNKFPHFKCEKCSFKENADYNAALNISNPKLKSTKEEP

SEQ ID NO: 2543 - protein, 726 aa, synthetic construct
SEVEFSHEYWMRHALTLAKRARDEREVPVGAILVLNNRVIGEGWNRAIGLHDPTAHAEIMALRQGGLVMQNYRLTDATLYVTFEPCVMCAGAMIHSRIGRVVFGVRNSKRGAAGSLMNVLSYPGMNHCVEITEGILVDECAALLCDFYRMPRQVLNAQKKAQSSISSGSSSGGSNGSETPGASESVTPKSSAGSSAGSTKNTITKTIKLRIVRPYNSAEVEKIVADEKDNREKIALEKNKDKVKEACSKHLKVAAYCTTQVERNACLFCKARKLDDKFYQKLKGQFPDAVFWQELGEIFRQLQKQAAEIYNQSLIELYYEIFIKGKGLANASSVEHYLSDVCYTRAAELFKNAAIASGLRGKVKSNFKLKELKSMKSGLPSTKSDNFPIPLVKQRGGQYTGFEISSHNDDFIIKIPFGRWQVKKEIDKYRPWEKFDFEQVRKSPKPISLLLSTQRRKRNKGWSKDEGTEAEIRKVMNGDYQTSYIEVKRGSKSGEKSAWVLNLSIDVPKIDKGVDPSIIGGIDVGVKSPLVCAINNAFSRYSISDNDLFRFNKKMFARRRILLKKNRHKRAGHGAKNKLKPISILTGKSERFRKKLIERWACEIADFFIKNKVGTVQMENLESMKRKEDSYFNIRLRGFWPYAEMQNKIEFKLKQYGIEIRRVAPNNTSRTCSKCGHLNNYFNFEYRKKNKFPPFKCEKCNFMENADYNAALNISNPKLKSTKEEP

SEQ ID NO: 2544 - protein, 726 aa, synthetic construct
SEVEFSHEYWMRHALTLAKRARDEREVPVGAILVLNNRVIGEGWNRAIGLHDPTAHAEIMALRQGGLVMQNYRLTDATLYATFEPCVMCAGAMIHSRIGRVVFGVRNSKHGAAGSLMNVLNYPGMNHRVEITEGILADECAGLLCDFYRMPRQVFSARKKAQSSINSSGSSGGSSGSETPGTSESATPESSGGGSSGSAKNTITKTLQLRIVRPYNSAEVEKIVADEKNNREKIALEKNKDKVKEACSKHLKVASYCTTQVERNACPFCKARKLDDKFYQKLRGQFPDAVFWQELSEILRQLQKQAAEVYNQSLIELYYEIFIKGRGFANASSVEHYLSDVCYTRAAELFKNAAIASGLRGKVKSNFRLKELKNMKSGLPTTKSDNFPIPLVKQKGGQYTGFEISSHNDDFIIKIPFGRWQVKKEIDKYRPWEKFDFEQVRKSPKPISLLLSTQRRKRNKGWSKDEGTEAEIRRVMNGDYQTSYIEVKRGSKIGEKSAWMLNLSIDVPKIDKGVDPSIIGGIDVGVKSPLVCAINNAFSRYSISDNDLFHFNKKMFARRRILLKKNRRRRAGHGAKNKLKPITILTEKSVRFRKKLIERWACEIADFFIKNKVGTVQMENLESLKGKEDSYFNIRLRGFWPYAEMQNKIELKLKQYGIKIRKVAPNNTSKICSKCGHLNDYFNFEYRKKNKFPHFKCEKCNFKEDADYNAALNISNPKLKSTKEEP

SEQ ID NO: 2545 - protein, 726 aa, synthetic construct
SEVEFSHEYWMRHALTLAKRARDEREVPVGAVLVLNNRVIGEGWNRAIGLHDPTAHAEIMALRQGGLVLQNYRLADATLYVTFEPCVMCAGAMIHSRIGRVVFGVRNSKHGAAGSLVNVLNYPGMNHRVEITEGILADECAALLCDFYRMPRQVFNARKKAQSNINSGGLSGGNSGSETPGASESATPESSGGGSSGSAKNTITKTLQLRIVRPYNSAEVEKIVADEKNNREKIALEKNKDKVKEACSKHLKVAAYCTTQVERNACLFCKARKLDDKFYQKLRGQFPDAVFWQEIGEIFRQLQKQAAEIYNQSLIELYYEIFIRGKGFANASSVEHYLSDVCYTRAAELFKNAAIASGLRGKVRSNFRLKELKNMRSGLPTTKSDNFPIPLVKQKGGQYTGFEISSHNGDFIIKIPFGRWQVKEETDKYRPWEKFDFEQVRKNPKPISLLLSTQRRKRNKGWSKDEGTEAEIRKVMNGDYQTSYVEVKRGSKIGEKSAWMLNLSIDVPKIDKGVDPSIIGGIDVGVKSPLVCAINNAFSRYSISDNDLFRFNKKMFARRRILLKKSKHKRAGHGAKNKLKPITILTEKSGRFRKKLIERWACEIADFFIKNKVGTVQMENLESMKRKEDSYFNIRLRGFWPYAEMQNKIEFKLKQYGIKIRKVAPNNTSKTCSKCGHLNNYFNFEFRKKNKFPHFKCEKCNFKEDADYNAALNISNPKLKSTKEEP

SEQ ID NO: 2546 - protein, 726 aa, synthetic construct
SEVEFSHEYWMRRALTLAKRARDEREVPVGAVLVLNNRVVGVGWNRAVGLHDPTAHAEIMALRQGGLVMQNYRLIEATLYVTFEPCIMCAGAMIHSRIGRVVFGARNSKRGAAGSLMNVLNYPGMNHRVEITEGILADECAALLCDYYRMPRQVFNARKKAQSSINSGGSSDGGSGSETPGTSESATPESSGGSSGGSAKNTITKTLKLRIVRPYNSAEVEKIVADEKNNREKIALEKNKDKVKEACSEHLKVAAYCTTQVGRNACLFCKARKLDDKFYQKLRGQFPDAVFWQELGEILRQLQKQAAEIYNQSLIELYYEIFIKGRGFANASSVEHYLSDVCYTRAAELFKNAAIASGLRGKVKSNFRLKELKNMKSGLPTTKSDNFPIPLVKQKGGQYTGFEISSHDDDFIIKIPFGRWQVKKEIDKYRPWEKFDFEQVRKSPKPISLLLSTQRRKRNKGWGKDEGTEAEIKKVMNGDYQTSYIEVKRGGKIGEKSAWMLNLSIDVPKIDKGVDPSIIGGIDVGVKSPLVCAINNAFSRYSISDNDLFRFNKKMFARRRILLKKSKHKRAGHGAKNKLKPITILTEKSGRFRKKLIERWACEIADFFIKNKVGTVQMENLESMKRREDSYFNIRLRGFWPYAKMLNKIEFKLKQYGIKIRKVAPNNTSKTCSKCGHLNNYFNFEYRKKNKFPHFKCEKCNFKENADYNAALNISNPKLKSTKEEP

SEQ ID NO: 2547 - protein, 726 aa, synthetic construct
SEVEFSHEYWMRHALTLAKRARDEREVPVGAVLVLNNRVIGEGWNRTTGLHDPTAHAEIMALRQGGLVMRNYRLTDATLYVTFEPCVMCAGAMIHSRIGRVVFGVRNSKRGAAGSLMNVLNCPGMNHCVEITEGILVDECAALLCDFYRMPRQVLNAQKKAQSSISPGGSSGGSSGSETPGASESVTPKSSGGSSGGSAKNTITKTLKLRIVRPYNSAEVEKIVADEKNNREKIALEKNKGKVKEACSKHLEVAAYCTTQVERNACLFCKARKLDDKFYQKLRGQFPDAVFWQELGEIFRQLQKQAAEIYNQSLIELYYEIFIKGRGFANASSVEHYLSDVCYTRAAELFKNAAIASGLRGKVKSNFRLKELKNMKSGLPTTKSDNFPIPLVKQKGGQYTGFEISSHNDDFIIKIPFGRWQVKKEIDKYRPWEKFDFEQVRKSPKPISLLLSTQRRKRNKGWSKDEGTEAEIRKVMNGDYQTSYIEVKRGSKTGEKSAWMLNLSIDVPKIDKGVNPSIIGGIDVGVKSPLVCAINNALSRYSISDNDLFRFNKKVFARRRILLKKNRHKRAGHGTKNKLKPITILTEKSGRFRKKLIERWACEIANFFIKNKVGTVQMENLESMKRKEDSYFNIRLRGFWPYAEMQNKIEFKLKQYGIKIRRVAPNNTSKTCSKCGHLNNYFSFEYRKKNKFPHFKCEKCNFKEDADYNAALNISNPKLKSTKEEP

SEQ ID NO: 2548 - protein, 726 aa, synthetic construct
SEVEFSHEYWMRHALTLAKRARDEREVPVGAILVLNNRVIGEGWNRAIGLNDPTAHAEIMALRQGGLVMQNHRLVDATLYVTFEPCVMCAGAMIHSRIGRVVFGVRNSKRGAAGSLTNVLNYPGMNHRVEITEGILVGECAALLCDFYRMPRQVFNARKKAQSSINPGGSSGGSSGSETPGTSENATPESSGGSSGSSAKNTITKTLKLRIVRPYNSAEVEKIVADEKNNREKIALEKNKDKVREACSKHLKVAAYCTTQVERDACLFCKARRLDDKFYQKLRGQFPDAVFWQEIGEIFRQLQKQAAEIYNQSLIELYYEIFIKGKGFANASSVEHYLSDVCYTRAAELFKNAAIASGLRGKVKSNFRLKELKNMKSGLPTTKSDNFPIPLVKQKGGQYTGFEISSHNDDFIIKIPFGRWQVKEEIDKYRPWEKFDFEQVRKSPKPISLLLSTQRRKRNKGWSKDEGTEAEIRKVMNGDYQTSYIEVKRGSKIGEKSAWMLNLSIDVPKIDKGVDPRIIGGIDVGVQSPLVCAINNAFSRYSISDNDLFHFNKKMFARRRILLKKNGHKRAGHGAKNKLKPITIMTEKSKRFRKKLIERWACEIADFFIKNKVGTVQMENLESMKRKEDSYFNVRLRGFWPYAEMQNKIEFKLKQYGIVVRKVAPNNTSKTCSKCGHLNNYFNFEYRKKNKFPHFKCEKCNFKENADYNAALNISNPKLKSTKEEP

SEQ ID NO: 2549 - protein, 726 aa, synthetic construct
SEVEFSHEYWMRHALSLAKRARDEREVPVGAVLVLNNRIIGEGWNRAIGLHDPTAHAEIMALRQGGLVMQNYRLTGATLYVTFEPCVMCAGAMVHSRIGRVVFGVRNSKRGAAGSLMNVLNYPGMNHCVEITEGILVDECAALLCDFYRMPRQVLNARKKARSNINSGGSSGGSSGSETLGTREGATPESSGGSSGGSAKNTITKTLKLRIVRPYNSAEVEKIVVDEKNNREKVALEKNKDKVKEACSEHLKVAAYCTTQVERSACLFCKARKLDDKFYQKLRGQFPDAVFWQELGGIFRQLQKQAAEIYNQSLIELYYEIFIKGKGITNASRVEHYLSDVCYTRAAELFKNAAIASGLRSKVRSNFRLKELKNMKSGLPTTKSDNFPIPLVRQKGGQYTGFEISNHDGDFIIKIPFGRWQVKKEINKHRPWEKFDFEQVRKSPKPISLLLSTQRRKRNKGWSKDEGTEAEIRKVMNGDYQTSYIEVKRGSKIGEKSAWMLSLSIDVPKIDKGVDPRIIGGIDVGVKSPLVCAINNASSRYSISDNDLFHFNKKMFARRRILLKKNRHKRAGHGAKNKLKPITILTEKSVRFRKKLIERWACEIADFFIKNKVGTVQMENLESMKGKEDSYFNIRLRGFWPYAEMQNKIEFKLKQYGIEIRKVAPNNTSKTCSKCGHLNNYFNFEYRKKNKFPYFKCEKCNFKENADYNAALNISNPKLKSTKGEP

SEQ ID NO: 2550 - protein, 726 aa, synthetic construct
SEVEFSHEYWMRHALTLAKRARDEREVPVGAVLVLNNRVIGEGWNRAIGLHDPTAHAEIMALRQGGLVMQNYRLTDATLYVTFEPCVMCAGAMVHGRIGRVVFGVRNSKRGAAGSLMNVLNYPGVNHCVEITEGILVDECAALLCDFYRMPRQVLNAQKKAQSSISPGGSSGGCSGSEMPGASESATPKSSGGSSAGSTKNAITKTLKLRIVRPYNSAEVEKIVADEKNNRERIALEKNKDKVKEACSKHLKVASYCTTQVERSACPFCKARKLDDKFYQKLGGQFPDAVFWQELGEIFRQLQKQAAEIYNQSLIELYYEIFIKGKGFANASSVEHYLSDVCYTRAAELFKNAAIASGLRGKVKSNFRLKELKNMKSGLPTTKSDNFPIPLVKQKGGQYTGFEISSHNDDFIIKIPFGRWQVKKEIDKYRPWEKFDFEQVRKSPKPISLLLSTQRRKRNKGWSKDEGTEAEIRKVMNGDYQTSYIEVKRGSKTGEKSAWMLNLSIDVPKIDKGVDPSIIGGIDVGVKSPLVCAINNAFSRYSISDNDLFRFNKKMFARRRILLKKNRHKRAGHGAKNKLKPISILTEKSKRFRKKLIERWACEIADFFIRNKVGTVQMENLESMKGKEDSYFNIRLRGFWPYAEMQSKIEFKLKQYGIEIRKVAPNNTSRTCSKCGHLNNYFNFEYRKKNKFPHFKCEKCYFKEDADYNAALNISNPRLKSTKEEP

SEQ ID NO: 2551 - protein, 726 aa, synthetic construct
SEVEFSHEYWMRHALTLAKRARDEHEVPVGAVLVLNNRVIGEGWNRAIGLHDPTAHAEIMALRQGGLVMQNYRLTDATLYVTFEPCVMCAGAMIHSRIGRVVFGVRNSKRGAAGSLMNVLNYPGMNHCVEITEGILVDECAALLCDFYRMPRQVLNAQKKAQSSISSGGSSGGSSGSETPGASESATPKSSSGSSASSTKNTITKTLKLRIVRPYNSAEVEKIVADEKSNREKIALEKNKDKVKEACSEHLKVAAYCTTQVERSACLFCKARKLDDKFYQKLRGQFPDAVFWQEIGEIFRQLQKQAAEIYNQSLIELYYEIFIKGKGFANASSVEHYLSDVCYTRAAELFKNAAIASGLRGKVKSNFRLKELKNMRSGLPTAKSDNFPIPLVKQKGGQYTGFEISSHNDDFIIKIPFGRWQVKKEIDKYRPWEKFDFEQVRKSPKPISLLLSTRRRKRNKGWSKDEGTEAEIRKVMNGDYQTSYIEVKRGSKIGEKSAWMLNLSIDVPKVDKGVDPSIIGGIDVGVKSPLVCAINNAFSRYSISDNELFHFNKKMFARRRILLKKNRHKRAGHGAKNKLKPISVLTEKSGRFRKKLIERWACEIADFFIKNKVGTVQMENLGSMKRKEDSYFNIRLRGFWPYAEMQNKIEFKLKQYGIEIRKVAPNNTSKTCSRCGHLNNYFNFEYRRENKFPHFKCEKCNFKENADYNAALNISNPKLKSTKEEP

SEQ ID NO: 2552 - protein, 726 aa, synthetic construct; identical to SEQ ID NO: 684

SEQ ID NO: 2553 - protein, 726 aa, synthetic construct
SEVEFSHEYWMRHALTLAKRARDEREVPVGAVLVLNNRVIGEGWNRAIGLNDPTAHAEIMALRQGGLVMQNYRLIDATLYVTFEPCVMCAGAMIHSRIGRVVFGVRNNKHGAAGSLVNVLNYPGMNHRVEITEGILADECAALLCDFYRMPRQVFNARKKAQSSINPGGSSGGSSGSETPGTSESATPESSGGSSGGSAKNTITKTLKLRIVRPYNSTEVEKIVADEKNNREKIALEKNKDKVKEACSEHLKVAAYCTTQVERNACLFCKARKLDDKFYQKLRGQFPDAVFWQEIGEIFRQLQRQAAEIYNQSLIELYYEIFIKGKGFANASSVEHYLSDVCYTRAAELFKNAAIASGLRGKVKSNFRLKELKNMKSGLPTTKSDNFPIPLVKQKGGQYTGFVISSQNDDFIIKIPFGRWQGKKEVDKYRPWEKFDFEQVRKSPKPISLLLSTQRRKRNKGWSKDEGTEAEIKKVMNGDYQTSYIEVKRGSRIGEKSAWMLSLSIDVPKIDRGVDPSIIGGIDVGVKSPLVCAINNASSRLSISDNDLFRFNKKMFARRRILLKKNGHKRAGHGAKNKLKPITILTEKSVRFRKKLIERWACEIADFFIRNKVGTVQMENLEGMKRKEDSYFNIRLRGFWPYAEMQNKIEFKLKQYGIEIRKVAPNNTSKTCSRCGHLNNYFSFEYRKKNKFPHFKCEKCNFKENADYNAALNISNPRLKSTKEEP

SEQ ID NO: 2554 - protein, 726 aa, synthetic construct
SEVEFSHEYWMRHALTLAKRARDGREVPVGAVLVLNNRVIGEGWNRAIGLHDPTAHAEIMALRQGGLVMQNYRLIDATLYVTFEPCVMCAGAMVHSRIGRVVFGVRNSKRGAAGSLMNVLDYPGMNHRVEITEGILADECAALLCDFYRMPRQVFNARKKAQSSISPGGSSGGSSGSETPGTSESATPESSGGSSGGSAKNTITKTLTLRIVRPYNSAEVEKIVADEKNNREKIALEKNKDKVKEACSRHLKVASYCTTQVERNACPFCKARKLDDKFYQKLRGQFPDAVFWQELGEILRQLQKQAAEIYNQSLIELYYEIFIKGRGFANDSSVEHYLSDVCYTRAAELFKNAAIASGLRGKVKSNFRLKELKNMKSGLPTTKSDNFPIPLVKQKGGQYTGFEISSHNDDFIIKIPFGRWQVKKEIDKYRPWEKFDFEQVRKSPKPISLLLSTQRRKRNKGWGKDEGTEAEIRKVMNGDYQTSYIEVKRGSKIGEKSAWMLNLSIDVPKIDKGVDPSIIGGIDVGVKSPLVCAINNALSRYSISDNDLFHFNKKMFARRRILLRKNRHKRAGHGARNKLKPISILTEKSGRFRKKLIERWACEIADFFIKNKVGTVQMENLESMKRKEDSYFNIRLRGFWPYAEMQNKIEFKLKQYGIEIRKVAPNNTSKTCSKCGHLNNYFNFEYRKRNKFPHFKCEKCNFKEDADYNAALNISNPKLKSTKEEP

SEQ ID NO: 2555 - protein, 726 aa, synthetic construct
SEVEFSHEYWMRHALTLAKRARDEREVPVGAILVLNNRVIGEGWNRAIGLHDPTAHAEIMALRQGGLVMQNYRLIDATLYVTFEPCVMCAGAMIHSRIGRVVFGVRNSKHGAAGSLMNVLNYPGMNHRVEITEGILADECAALLCDFYRMPRQVFNARKKAQSSINPGGPSGGSSGSETPDTSESATPESSGGNSGGSAKNTITKTLKLRIVRPYNSAEVEKIVADEKYNREKIALEKNKNKVREACSEHLKVAAYCTTQVERSACLFCKARKLDDKFYQKLRGQFPDAVFWQETGEIFRQLQRQAAEIYNQSLIELYYEIFIKGKGFANASSVEHYLSDVCYTRAAELFKNAAIASGLRGKVKSNFRLKELKNMKSGLPTTKSDNFPIPLVKQKGGQYTGFEISSHNDDFIIKIPFGRWQVKKEIDKYRPWEKFDFEQVRKSPKPISLLLSTQRRKRNKGWSKDEGTEAEIRKVMNGDYQTSYIEVKRGSKTGEKSAWMLNLSIDVPKIDKGVDPSIIGGIDVGVKSPLVCAINNAFSRYSISDNDLFRFNKKMFARRRILLKKNRHKRAGHGAKNKLKPTSILTEKSRRFRKKLIERWACEIADFFIKNKVGTVQMENLEGMKRREDSYFNIRLRGFWPYAEMQNKIEFKLKQYGIEIRKVAPNNTSKTCSKCGHLNNHFNFEYRRRNKFPHFKCEKCNFKENADYNAALNISNPKLKGTKEGP

SEQ ID NO: 2556 - protein, 726 aa, synthetic construct
SEVEFSHEYWMRHALTLAKRARDEREVPVGAVLVLNNRVIGEGWNRAIGLHDPTAHAEIMALRQGGLVMQNYRLTDATLYVTFEPCVMCAGAMIHSRIGRVVFGVRNSKHGAAGSLVNVLNYPGMNHRVEITEGVLADECAALLCDFYRMPRQVFNARKKAQSNINPGGSSGGSSGSETPGTSDSATPGSSGGSSGGSAKNTITKTLKLRIVRPYNSAEVEKIVADEKNNREKIALEKNKDKVREACSKHLKVASYCTTQVERNACPFCKARKLDDKFYQKLRGQFPDAVFWQELGEILRQLQKQAAEIYNQSLIELYYEIFIKGRGFANASSVEHYLSDVCYTRAAELFKNAAIASGLRGKVKGNFRPKELKNMKSGLPTTKSDNFPIPLVKQKGGQYTGFEISSHNDDFIIKIPFGRWQVKKEIDKYRPWEKFDFEQVRKSPKPISLLLSTQRRKKNKGWSKDEGTEAEIRRVMNGDYQTSYIEVKRGSKIGEKSAWMLNLSIDVPTIDKGVDPSIIGGIDVGVKSPLVCAINNSSSRYSICDNDLFRFNKKMFARRRILLKKNRHKRAGHGTKNKLKPITILTKKSERFRKKLIERWVCEVADFFIKNEVGTVQMENLESMKRREDSYFNIRLRGFWPYAEMQNRIELKLKQYGIEIRRVAPNNTSRTCSKCGHLNNYFNFEYRKKNKFPHFKCEKCNFREDADYNAALNISNPKLKSTKEEP

SEQ ID NO: 2557 - protein, 726 aa, synthetic construct
SEVEFSHEYWMRHALTLAKRARDEREVPVGAILVLNNRVIGVGWNRAIGLHDPTAHAEIMALRQGGLVMRNYRLVDATLYVTFEPCVLCAGAMVHSRIGRVVFGVRNSKRGAAGSLMNVLNYPGMNHRVEITEGILADECAALLCDFYRMPRQVFNARKRARSNINSGGPSGGSSGSETPSTSESATPESSGGGFGGSAKNTITKTLQLRIVRPYNSAEVEKIVADEKNNREKIALEKNKDKVKEACSKHLKVASYCTTQVERNACLFCKARKLDDKFYQKLRGQFPDAVFWQEIGEIFRQLQKQAAEIYNQSLIELYYEIFIKGKGFANASSVEHYLSDVCYARAAELFKNAAIASGLRGKVKSNFRLKELKNMKSGLPTTKSDNFPIPLVKQKGGQYTGFEISSHNDDFIIKIPFGRWQVKKEIDKYRPWEKFDFEQVRKSPKPISLLLSTQRRKRNKGWSKDEGTEAEIRKVMNGDYQTSYIEVKRGSKIGEKSSWMLSLSIDVPKIDKGVDPSIIGGIDVGVKSPLVCAINNALGRYSISDNDLFHFNKKMFARRRILLKKNRHKRAGHGAKNKLKPLTILTKKSGRFRKKLIERWACEIANFFIKNKVGTVQMENLESMKRKEDSYFNIRLRGFWPYAEMQNKIEFKLKQYGIKIRKVAPNNTSKTCSKCGHLNNYFGFEYRRKNKFPHFKCEKCNFKEDADYNAALNISNPKLKSTREEP

SEQ ID NO: 2558 - protein, 726 aa, synthetic construct
SEVEFSHEYWMRHALTLAKRARDEREVPVGAVLVLNNRVIGEGWNRTTGLHDPTAHAEIMALRQGGLVMQNHRLVDATLYVTFEPCVMCAGAMIHSRIGRVVFGVRNSKRGAAGSLMNVLNYPGMNHCVEITEGILVDECAALLCDFYRMPRQVLNAQKKAQSSISSGGSSGGSSGSETPGASGSVTPKSSGGSSAGSTKDTITKTLKLRIVRPYNSAEVEKVVADEKNNRERIALEKNKDKVKEACSKHLKVAAYCTTQVERNACLFCKARKLDDKFYQKLRGQFPDAVFWQEIGEIFRQLQRQAAEIYNQSLIELYYEIFIKGKGFANASSVEHYLSDVCYTRAAELFKNAAIASGLRGKVKSNFRLKELKNMKSGLPTTKSDNFPIPLVKQKGGQYTGFEISSHNGDFIIKIPFGRWQVKKEIDKYRPWEKFDFEQVRKSPKPISLLLSTQRRRRNKGWSKDEGTEAEIRKVMNGDYQTSYIEVKRGSKIGEKSAWMLSLSIDVPKIDKGVDPSIIGGIDVGVKSPLVCAINNAFCRYSISDNDLFHFNKKMFARRRILLKKSRHKRAGHGAKNKLKPISILTEKSKRFRKKLIERWACEIADFFIKNKVGTVQMENLESMKRKEDSYFNIRLRGFWPYAKMQNKIEFKLKQYGIEIRKVAPNNTSKTCSKCGHLNNYFNFEYRKKNKFPHFKCEKCNFKESADYNAALNISNPKLKSTKEEP

SEQ ID NO: 2559 - protein, 726 aa, synthetic construct
SEVEFSHEYWMRHALTLAKRARDEREVPVGAILVLNNRVIGEGWNRAIGLHDPTAHAEIMALRQGGLVMQNYRLIDATLYVTFEPCVMCAGAMIHSRIGRVVFGVRNNKHGAAGSLVNVLNYPGMNHRVEITEGILADECAALLCDFYRMPRQVFNARKKAQSSINPGGSSGGSSGSETPGTSESATPESSGGSSGSSAKNTITKTLKLRIVRPYNSAEVEKIVADEKNSREKIALERNKDKVKEACSKHLKVAAYCTTQVERNACLFCKARKLDDKFYQELRGQFPDAVFWQEIGEIFRQLQKQAAEIYNQSLIELYYEIFIKGKGFANASSVEHYLSDVCYTRAAELFKNAAIASGLRGKVKSNLRLKELKNMKSGLPTTKSDNFPIPLVKQKGGQYTGFEISSHNDDFIIKIPFGRWQVKKEIDKYRPWEKFDFEQVRKSPKPISLLLSTQRRRRNKGWSKDEGTEAEIRKVMYGDYQTSYIEVKRGSKIGEKSAWMLNLSIDVPKIDKGVDPSIIGGIDVGVKSPLVCAINNALSRYSISDNDLFHFNKKMFARRRILLRKNRHKRAGHGARNKLKPITVLTEKSERFRKKLIERWACEIANFFIKNKVGTVQMENLESMKRREDSYFNIRLRGFWPYAEMQSKIEFKLKQYGIEVRKVAPNNTSKTCSKCGHLNNYFNFEFRKKNKFPHFRCEKCNFKEDADYNAALNISNPKLKSTKEEP

SEQ ID NO: 2560 - protein, 726 aa, synthetic construct
SEVEFSHEYWMRHALTLAKRARDEREVPVGAILVLNNRVIGEGWNRAVGLHDPTAHAEIMALRQGGLVMQNCRLIEATLYVTFEPCIMCAGAMIHSRIGRVVFGVRNSKRGAAGSLMNVLNYPGMNHRVEITEGILADECAALLCDYYRMPRQVFNARKKAQSSINSGGSSDGGSGSETLGTCESVTPESSGGSSGGSAKNTITKTLKLRIVRPYNSAEVEKIVADEKNNREKIALEKNKDKVKEACSEHLKVAAYCTTQVERSACLFCKARKLDDKFYQKLRGQFPDAVFWQEIGEIFRQLQKQAAEIYNQSLIELYYEIFIKGKGFANASSVEHYLSDVCYTRAAELFKNAAIASGLRGKVKSNFRLKELKNMKSGLPTTKSDNFPIPLVKQKGGQYTGFEISSHNDDFIIKIPFGRWQAKKEIDKYRPWEKFDFEQVRKSPKPISLLLSTQRRKRNKGWSKDEGTEAEIRKVMNGDYQTSYIEVKRGSKIGEKSAWMLNLSIDVPKIDKGVDPSIIGGIDVGVKSPLVCAINNAFSRYSISDNDLFRFNKKVFARRRILLKKSKHKRAGHGAKNKLKPITILTEKSGRFRKKLIERWACEIADFFIKNKVGTVQMENLEGMKRKEDSYFNIRLRGFWPYAEMQNKIEFKLKQYGIEIRKVAPNNTSKTCSKCGHLNNYFNFEYRKKNKFPHFKCEKCNFKENADYNAALNISDPKLKSTKEEP

SEQ ID NO: 2561 - protein, 726 aa, synthetic construct
SEVEFSHEYWMRHALTLAKRARDEREVPVGAVLVLNNRVIGEGWNRAIGLHDPTAHAEVMALRQGGLVMQNYRLTDATLYVTFEPCVMCAGAMIHSRIGRVVFGVRNSKRGAAGSLMNVLNYPGMNHRVEITEGILADECAALLCDFYRMPHQVFSARKKAQSSINPGGSSGGSSGSKTPGTSESATPESSGGSSGGSAKNSITKTLKLRIVRPYNSAEVEKIVADEKNNREKIALEKNKGKVKEACSKHLKVATYCTTQVERNACLFCKARKLDDKFYQKLRGQFPDAVFWQEIGEIFRQLQKQAAEIYNQSLIELYYEIFIEGKGFANASSVEHYLSDVCYTRAAELFKNAAIASGLRGKVKGNFRLKELKSMKSGLPTTKSDNFPIPLVKQKGGQYTGFEISSHNDDFIIKIPFGRWQVKKEIDKYRPWEKFDFEQVRKSPKPISLLLSTRRRKRNKGWSKDEGTEAEIRKVMNGDYQTSYIEVKRGSKIGEKSAWMLNLSIDVPKIDKGVDPSIIGGIDVGVKSPLVCAINNAFSRYSISDNELFHFNKKMFARRRILLKKNRHKRAGHGAKNKLKPITILTEKSRRFRKKLIERWACEIADFFIKNKVGTVQMESLESMKRKEDSYFNIRLRGFWPYAEMQNKIEFKLKQYGIKIRKVAPNNTSKTCSMCGHLNNYFSFEYRKKNKFPHFKCEKCNFKENADYNAALNISNPKLMSTKEGP

SEQ ID NO: 2562 - protein, 726 aa, synthetic construct
SEVEFSHEYWMRHALILAKRARDEREVPVGAVLVLNNRVIGVGWNRAIGLHDPTAHAEIMALRQGGLVMQNYRLIDATLYVTFEPCVMCAGAMIHSRIGRVVFGVRNSKHGAAGSLVNVLNYPGMNHRVEITEGILADECAALLCDYYRMPRQVLNARKKAQSSVSSGGSSGGSSGSETPGASGSVTPKSSVGSSAGSTKNTITKTLKLRIVRPYNSAEVEKIVADEKNNREKIALEKNKDKVKEACSEHLKVAAYCTTQVERSACLFCKARKLDDKFYQKLRGQFPDAVFWQEIGEIFRQLQKQAAEIYNQSLIELYYEIFIKGKGFANASSVEHYLSDVCYTRAAELFKNAAIASGLRGKVKSNFRLKELKNMKSGLPTTKSDNFPIPLVKQKGGQYTGFEINSHNDDFIIKIPFGRWQVKKEIDKYRPWEKFDFEQVRKGPKPISLLLSTRRRKRNKGWSKDEGTEAEIRKVMNGDYQTSYIEVKRGSKTGEKSAWMLNLSIDVPKIDKGVDPSIIGGIDVGVKSPLVCAINNAFSRYSISDNDLFRFNKKMFARRRILLKKNRHKRAGHGAKNKLKPISILTGKSERFRRKLIERWACEIADFFIKNKVGTVQMENLESMKRKEDSYFNIRLRGFWPYAEMQNRIEFKLKQYGIEIRKVAPNNTSKTCSKCGHLNNYFNFEYRKKNKFPHFKCEKCNFKENADYNAALNISNPKLKSTKEEP

SEQ ID NO: 2563 - protein, 726 aa, synthetic construct
SEVEFSHEYWMRHALTLAKRASDEREVPVGAILVLNNRVIGEGWNRAIGLHDPTAHAEIMALRQGGLVMQNYRLIDATLYVTFEPCVMCAGAMIHSRIGRVVFGVRNNKHGAAGSLVNVLNYPGMNHRVEITEGILADECAALLCDFYRMPRQVFNARKKAQSSINPGGSSGGSSGSETPGTSESATPESSGGSSGSSAKNTITKTLKLRIVRPYNSAEVEKIVADEKNSREKIALEKNKDKVKEACSKHLKVAAYCTTQVERNACLFCKARRLDDKFYQKLRGQFPDAVFWQELGEIFRQLQKQAAEIYNQSLIELYYEIFIKGRGFANASSVEHYLSDVCYTRAAELFKNAAIASGLRGKVKSNFRLRELKNMKSGLPTTKSDNFPIPLVKQKGGQYTGFEISSHNDDFIIKIPFGRWQVKKEIDKYRPWEKFDFEQVRKSPKPISLLLSTQRRKKNKGWSKDEGTEAEIRRVMNGDYQTSYIEVKRGSKIGEKSAWMLNLSIDVPKIDKGVDPSIIGGIDVGVKSPLVCAINNSSSRYSICDNDLFRFNKKMFARRRILLKKSKHKRAGHGAKNKLKPITILTGKSRRFRKKLIERWACEIADFFIKNKVGTVQMENLEGMKRKEDSYFNIRLRGFWPYAEMQNKIEFKLKQYGIEIRKVAPNNTSKTCSKCGHLNNYFNFEYRKKNKFPHFKCEKCSFKENADYNAALNISNPKLKSTKEEP

SEQ ID NO: 2564 - protein, 726 aa, synthetic construct
SEVEFSHEYWMRHALTLAKRARDEREVPVGAILVLNNRVIGEGWNRAIGLHDPTAHAEIMALRQGGLVMQNYRLIDATLYVTFEPCVMCAGAMIHSRIGRVVFGVRNNKHGAAGSLVNVLNYPGMNHRVEITEGILADECAALLCDFYRMPRQVFNARKKARSNINSGGSSGGSSGSETPGTSESAAPESSGGSSGGSTRNTITKTLKLRIVRPYNSAEVEKIVADEKNNREKIALEKNKGKVKEACSKHLKVATYCTTQVERNACLFCKARKLDDKFYQKLRGQFPDAVFWQEIGEIFRQLQKQAAEIYNQSLIELYYEIFIEGKGFANASSVEHYLSDVCYTRAAELFKNAAIASGLRGKVKSNFRLKELKNMKSGLPTTKSDNFPIPLVKQKGGQYTGFEISSHNDDFIIKIPFGRWQVKKEIDKFRPWEKFDFEQVRKSPKPISLLLSTQRRKRNKGWSKDEGTEAEIRKVMNGDYQTSYIEVKRGSKIGEKSAWMLSLSIDVPKIDKGVDPSIVGGIDVGVRSPLVCAINNALGRYSISDNDLFHFNKKMFARRRILLKKSKHKRAGHGAKNKLKPITILTEKSRRFRKKLIERWACEIADFFIRNKVGTVQMENLESMKRKEDSYFNIRLRGFWPYAEMQNKIEFKLKQYGIEIRKVAPNNTSKTCSKCGHLNNYFNFEYRKKNKFPHFKCEKCNFKENADYNAALNISNPMLKSTKEEP

SEQ ID NO: 2565 - protein, 726 aa, synthetic construct
SEVEFSHEYWMRHALTLAKRARDEREVPVGAVLVLNNRVIGEGWNRAIGLHDPTAHAEIMALRQGGLVMQNYRLTDATLYVTFEPCVMCAGAMIHSRIGRVVFGVRNSKRGAAGSLMNALNYPGMNHCVEITEGILVDECAALLCDFYRMPRQVLNAQKKAQSSISSGGSSGGSSGSETPGASESATPESSGGSSSGSTKNTITKTLKLRIVRPYNSTEVEKIVADEKNNREKIALEKNKDKVKEACREHLKVASYCTTQVERNACLFCKARKLDDKFYQKLRGQFPDAVFWQELGEIFRQLQKQAAEIYNQSLIELYYEIFIKGKGLANASSVEHYLSDVCYTRAAELFKNAAIASGLRNKIKSNFRLKELKSMKSGLPTTKSDNFPIPLVKQKGGQYAGFEISSHNDDFIIKIPFGRWQVKKEIDKYRPWEKFDFEQVRKSPKPISLLLSTRRRKRNKGWSKDEGTEAEIRKVMNGDYQTSYIEVKRGSKIGEKSAWMLNLSIDVPKVDKGVDPCIIGGIDVGVKSPLVCAISNAFSRYSISDNDLFHFNKKMFARRRILLKKNRHKRAGHGAKNKLKPISILTEKSKRFRKKLIERWACEIADFFIKNKVGTVQMENLESMKRREDSYFNIRLRGFWPYAEMQNKIEFKLEQYGIEIRKVAPNNTSRTCSKCGHLNNYFNFEYRKKNKFPHFKCEKCNFKENADYNAALNISNPKLKSTKEEP

SEQ ID NO: 2566 - protein, 726 aa, synthetic construct
SEVEFSHEYWMRHALILAKRARDEREVPVGAVLVLNNRVIGVGWNRAIGLHDPTAHAEIMALRQGGLVMQNYRLIDATLYVTFEPCAMCAGAMIHSRIGRVVFGVRNSKRGAAGSLMNVLNYPGMNHRVEITEGILADECAALLCDYYRMPRQVFNARKKAQSSINSGGSSGGSSGSVTPGPSESATPESSGGSSGSSAKNTITKTLQLRIVRPYNSAEVEKIVADEKNNREKIALEKNKDKVKEACSKHLKVASYCTTQVERNACLFCKARKLDDRFYQKLRGQFPDAVFWQETGEIFRQLQRQAAEIYNQSLIELYYEIFIKGKGFANASSVEHYLSDVCYTRAAELFKNAAIASGLRGKVKSNFRLKELKNMKSGLPTTKSDNFPIPLVKQKGGQYTGFEISSHNDDFIIKIPFGRWQVKKEIDKYRPWEKFDFEQVRKSPKPISLLLSTQRRKRNKGWSKDVGTEAEIRKVMNGDYQTSYIEVKRGSKIGEKSAWMLSLSIDVPKIDKGVDPSIIGGIDVGVKSPLVCAINNAFCRYSISDNDLFHFNKKMFARRRILLKKNRHKRAGHGAKNKLKPISILTGKSERFRKKLIERWACEIANFFIKNKVGTVQMENLESMKRREDSYFNIRLRGFWPYAEMQSKIEFKLKQYGIKIRKVAPNNTSKTCSKCGHLNNYFNFEYRKKSKFPHFKCEKCNFREDADYNAALNISNPKLKSTKEEP

SEQ ID NO: 2567 - protein, 726 aa, synthetic construct
SEVEFSHEYWMRHALTLAKRARDEREVPVGAVLVLNNRVIGEGWNRAIGLHDPTAHAEIMALRQGGLVMQNYRLVDATLYVTFEPCVLCAGAMVHSRIGRVVFGVRNSKRGAAGSLMNVLNYPGMNHRVEITEGILADECAALLCDFYRMPRQVFNARKKARSNINSGGSSGGSSGSEMPGTSESATPESSGGSSGGSAKNTITKTLKLRIVRPYNSAEVEKIVADEKNNREKIALEKNKDKVKEACSEHLKVAAYCTTQVERNACLFCKARKLDDRFYQKLRGQFPDAVFWQEVGEIFRQLQRQAAEIYNQSLIELYYEIFIKGKGFANASNVEHYLSDVCYTRAAELFRNAAIASGLRGKVKSNFRLKELKNMKSGLPTTKSDNFPIPLVKQKGGQYTGFEISSHNDDFIIKIPFGRWQAKKEIDRYRPWEKFDFEQVRKNPKPISLLLSTRRRKRNKGWSKDEGTEAEIRRVMNGDYQTSYIEVKRGSKIGEKSAWMLSLSIDVPKIDKGVDPSIIGGIDVGVKSPLVCAINNAFNRYSISDNNLFHFNKKMFARRRILLKKNRHKRAGHGAKNKLKPITILTEKSGRFRKKLIERWACEIADFFVKNKVGTVQMENLESMKRKEDSYFNIRLRGFWPYAEMQNKIEFKLKQYGIEIRKVAPNNTSKTCSKCGHLNNYFNFEYRRKNKFPHFKCEKCNFKENADYNAALNISNPKLKSTKEEP

SEQ ID NO: 2568 - protein, 726 aa, synthetic construct
SEVEFSHEYWMRHALTLAKRARDEREVPVGAVLVLNNRVIGGGWNRAIGLHDPTAHAEIMALRQGGLVMQSCRLVDATLYVTFEPCVMCAGAMIHSRIGRVVFGVRNSKRGAAGSLMNVLNYPGMNHRVEITEGILAGECAALLCDFYRMPRQVFNAQKKAQSTINSGGSSGGSSSSETPGTSGSATPEGSGGSSGGSAKNTITKTLKLRIVRPYNSAEVEKIVADEKNNREKIALEKNKDKVKEACSKHLKVASYCTTQVERNACLFCKARKLDDKFYQKLRGQFPDAVFWQELGEIFRQLQKQAAEIYNQSLIELYCEIFIKGKGFANASSVEHYLSDVCYTRAAELFKNAAIASGLRGKVKSNFRLKELKNMKSGLPTTKSDNFPIPLVKQKGGQYTGFEISSHNDDFIIKIPFGRWQVKKEIDKYRPWEKFDFEQVRKSPKPISLLLSTQRRKRNKGWSKDEGTEAEIRKVMNGDYQTSYIEVKRGSKIGEKSAWMLNLSIDVPKIDKGVDPSIIGGIDVGVKSPLVCAINNAFSRYSIGDNDLFHYNKKMFARRRILLKKNRHKRAGHGAKNKLKPISILTEKSKRFRKKLIERWACEIADFFIKNKVGTVQIENLESMKRKEDSYFNIRLRGFWPYAEMQNKIEFKLKQYGIEIRKVAPNNTSKTCSKCGHLNSYFNFEYRKKNKFPHFKCEKCNFKENADYNAALNISNPKLKSTKEEP

SEQ ID NO: 2569 - protein, 726 aa, synthetic construct
SEVEFSHEYWMRHALTLAKRARDEREVPVGAVLVLNNRVIGEGWNRAIGLHDPTAHAEIMALRQGGLVMQNYRLIDATLYVTFEPCVMCAGAMIHSRIGRVVFGVRNSKHGAAGSLVNVLNYPGMNHRVEITEGILADECAALLCDFYRMPRQVFNARKKAQSSINPSGSSGGSSGSVTPGTSESATPESSGGGFGGSAKNTITKTLQLRIVRPYNSAEVEKIVADEKNNREKIALEKNKDKVKEACSKHLKVASYCTTQVERNACLFCKARKLDDKFYQKLRSQFPDAVFWQELGEIFRQLQKQAAEIYNQSLIELYYEIFIKGKGFANASSVEHYLSDVCYTRAAELFKNAAIASGLRSKVRSNFRLKELKNMKSGLPTTKSDNFPIPLVKQKGGQYTGFEISSHNSDFIIKIPFGRWQEKEEIDKYRPWEKFDFEQVRKSPKPISLLLSTQRRKRNKGWSKDEGTEAEIRKVMNGDYQTSYIEVKRGSKIGEKSAWMLNLSIDVPKIDKGVDPSIVGGIDVGVKSPLVCAIDNVLSRYSISDNDLFHFNKKMFARRRILLKKNRHRRAGHGAKNKLKPISILTEKSKRFRKKLIERWACEIADFFIKNKVGTVQMENLESMKRKEDSYFNIRLRGFWPYAEMQNKIEFKLKQYGIEIRKVAPNNTSKTCSKCGHLNNYFSFEYRKKNKFPHFKCEKCNFKENADYNAALNISNPKLKSTKEEP

SEQ ID NO: 2570 - protein, 726 aa, synthetic construct
SEVEFSHEYWMRHALALAKRARDEREVPVGAILVLNNRVIGEGWNRAIGLHDPTAHAEIMALRQGGLVMQNHRLIDATLYVTFEPCVMCAGAMIHSRIGRVVFGVRNNKHGAAGSLVNVLDYPGMNHRVEITEGILADECAALLCDFYRMPRQVFNARKKAQSSISPGGSSGGSSGSETPGTSESATPESSGGSSGGSAKNTITKTLKLRIVRPYNCAEVEKIVADEKNNREKIALEKNKDKVKEACSKHLKVAAYCTTQVERNACLFCKARKLDDKFYQKLRGQFPDAVFWQEIGEVFRQLQKQAAEIYNQSLIELYYEIFIKGKGFANASSVEHYLSDVCYTRAAELFKNAAIASGLRGKVKSNFRLKELKNMKSGLPTTKSDNFPIPLVKQKGGQYTGFEISSHNDDFIIKIPFGRWQVKKEIDKYRPWEKFDFEQVRKSPKPISLLLSTQRRKRNRGWSKDVGTEAEIRKVMNGDYQTSYIEVKRGSKIGEKSAWMLNLSIDVPKIDKGVDPSIIGGIDVGVKSPLVCAINNAFSRYSISDNDLFHFNKKMFARRRILLKKTRHKRAGHGAKNKLKPISILTEKSERFRKKLIERWACEIADFFIKNKVGTVQMENLESMKRREDSYFSTRLRGFWPYAKMQNKIEFKLKQYGIEIRKVAPNNTSKTCSKCGHLNNYFNFEYRKKNKFPHFKCEKCNFKENADYNAALNISNPKLKSTKEEP

SEQ ID NO: 2571 - protein, 726 aa, synthetic construct
SEVEFSHEYWMRHALTLAKRARDEREVPVGAVLVLNNRVIGVGWNRAIGLHDPTAHAEIMALRQGGLVMQDYRLVDATLYVTFEPCVLCAGAMVHSRIGRVVFGVRNSKRGAAGSLMNVLNHPGMNHRVEITEGILADECAALLCDFYCMPRQVFNAQKRAQSSINSGGSSGGSSGSETPGTSESATPGSSGGSSGGSAKNTITKTLKLRIVRPYNSAEVEKIVADEKNNREKIALEKNKDKVKEACSKHLKVAAYCTTQVERNACLFCKARRLDDKFYQKLRGQFPDAVFWQEIGEIFRQLQKQAAEIYNQSLVELYYEILIKGKGIANASSVEHYLSDVCYTRAAKLFKNAAIASGLRNKIKSNFRLKELKNMKSGLPTTKSDNFPIPLVKQKGGQYTGFEISNHNGDFIIKIPFGRWQAKKEIDKYRPWEKFDFEQVRKSPKPISLLLSTQRRKRNRGWSRDEGTEAEVKKVMNGDYQISYIEVKRGSKIGGKSAWMLSLSIDVPKTDKGADPSIVGGIDVGVKSPLVCAINNALGRYSISDNDLFHFNKKMFARRRILLKKNRHKRAGHGARNKLKPITVLTEKSERFRKKLIERWACEIANFFIKNKVGTVQMENLESMKRKEDSYFNIRLRGFWPYAEMQNKIEYKLKQYGIEIRRVAPNNTSRTCSKCGHLNNYFNFEYRRKYKFPHFKCEKCNFKEDADYNAALNISNPKLKSTKEEP

SEQ ID NO: 2572 - protein, 726 aa, synthetic construct
SEVEFSHEYWMRHALTLAKRARDEREVPVGAVLVLNNRVIGVGWNRAIGLHDPTAHAEIMALRQGGLVLQNYRQTDATLYVTFEPCVMCAGAMIHSRIGRVVFGVRNSKRGAAGSLMNVLNYPGMNHRVEITEGILADECAALLCDFYHMPRRVFNAQKKAQSSINSGGSSGGSSGSETPGTSESPTPESSGGSSGSSAKNTITKTLQLRIVRPYNSAEVEKIVADEKNNREKIALEKNKDKVKEACSKHLKVAAYCTTQVERNACLFCKARKLDDKFYQKLRGQFPDAVFWQEIGEIFRQLQKQAAEIYNQSLIELYYEIFIKSKGFANASSVEHYLSDVCYTRAAELFKNAAIASGLRGKVKSNFRLKELRNMKSGLPTTKSDNFPIPLVRQKGGQYTGFEISNHNGDFIIKIPFGRWQVKKEINKHRPWEKFDFEQVRKSPKPISLLLSTQRRKGNKGWSKDEGTEAEIRKVMNGDYQTSYIEVKRGSKIGEKSAWMLNLSIDVPKIDKGVDPSIIGGIDVGVKSPLVCAVNNALSRYSISDNDLFHFNKKMFARRRILLRKNRHKRAGHGARNKLRPITVLTEKSERFRKKLIERWACEIANFFIKNKVGTVQMENLESMKRREDSYFNIRLRGFWPYAEMQSKIEFKLKQYGIEIRKVAPNNTSKTCSKCGHLNNYFNFEYRKKNKFPHFKCEKCNFKENADYNAALNISNPKLKSTKEEP

SEQ ID NO: 2573 - protein, 726 aa, synthetic construct
SEVEFSHEYWMRRALTLAKRARDEREVPVGAVLVLNNRVIGVGWNRAIGLHDPTAHAEIMALRQGGLVMQNYRLTDATLYVTFEPCVMCAGAMIHSRIGRVVFGVRNSKRGAAGSLMNVLNYPGINHCVEITEGILVDECAALLCDFYRMPRQVLNAQKKAQSSISSGGSSGGSSGSETPGSSESAAPESSGGGSSGSAKNTITKTLQLRIVRPYNSAEVEKIVADEKNNREKIALEKNKDKVKEACSKHLKVASYCTTQVERSACPFCKARKLDDKFYQKLRGQFPDAVFWQEIGEIFKQLQKQAAVIYNQSLIELYYEIFIKGKGIANASSVEHYLSDVCYTRAAELFKNAAIASGLRNKVKSNFRLKELKSMKSGLPTTKSDNFPIPLVRQKGGQYTGFEISNHNSDFIIKIPFGRWQAKKEIDKYRPWEKFDFEQVRKSPKPISLLLSTQRRKRNRGWSKDESTEAEIRKVMNGDYQTSYIEVKRGSKVGEKSAWMLNLSIDVPKIDKGVDPSIIGGIDVGVKSPLVCAINNAFSRYSISDNDLFHFNKKVFARRRILLKKNRHKRAGHGAKNKLKPISILTGKSERFRKKLIERWACEIADFFIKNKVGTVQMENLESMKRREDSYFNIRLRGFWPYAKMQNKIEFKLKQYGIEIRKVAPNNTSKTCSKCGHLNNYFNFEYRKKNKFPHFKCEKCNFKENADYNAALNISNPKLKSTKEEP

SEQ ID NO: 2574 - protein, 726 aa, synthetic construct
SEVEFSHEYWMRHALTLAKRARDEREVPVGAVLVLNNRVIGEGWNRAIGLHDPTAHAEIMALRQGGLVMQNHRLIDATLYVTFEPCVMCAGAMIHSRIGRVVFGVRNSKRGAAGSLMNVLNYPGMNHRVEITEGILADECAALLCDFYRMPRQVFNAQKKAQSSINSGGSSGGSSGSETPGTSESATPESSGGSPGGSAKNTITKTLKLRIVRPYNSAEVEKIVADEKNNREKIALEKNKDKVKEACSEHLKVAAYCTTQVERSACLFCKARKLDDKFYQKLRGQFPDAVFWQEIGEIFRQLQKQAAEIYNQSLIELYYEIFIKGKGFANASSVEHYLSDVCYTRAAELFKNAAIASGLRGKVKSNFRLKELKNMRSGLPTAKSDNFPIPLVKQKGGQYTGFEISSHNDDFVIKIPFGRWQVKKEIDKYRPWEKFDFEQVRKSPKPISLLLSTQRRKKNRGWSKDEGTEAEIKKVMNGDYQTSYIEVKRGSKIGEKSAWMLNLSIDVPKIDKGVDPSIIGGIDVGVKSPLVCAISNAFSRYSISDNDLFHFNKKMFARRRILLKKSKHKRAGHGAKNKLKPITILTEKSRRFRKKLIERWACEIADFFIKNKVGTVQMENLESMKRREDSYFNIRLRGFWPYAEMQNKIEFKLKQYGIEIRKVAPNNTSKTCSKCGHLNNYFNFEYRKKNKFPHFKCEKCYFKEDADYNAALNISNPKLRSTKEEP

SEQ ID NO: 2575 - protein, 726 aa, synthetic construct
NEDEFSHEYWMRHALTLAKRARDGREVPVGAVLVLNNRVIGEGWNRAIGLHDPTAHAEIMALRQGGLVMQNYRLIDATLYVTFEPCVMCAGAMVHSRIGRVVFGVRNSKRGAAGSLMNVLDYPGMGHRVEITEGILADECAALLCDFYCMPRQVFNAQKRAQSSINSGGSSGGSSGSETQGTSESATPESSGGGPSGSAKNTITKTLQLRIVRPYNSAEVEKIVADEKNNREKIALEKSKDKVKEACSKHLKVASYCTTQVERNACPFCKARKLDDKFYQKLRGQFPDAVFWQELGEIFRQLQKQAAEIYNQSLIELYYEIFIKGKGFANASSVEHYLSDVCYTRAAELFKNAAIASGLRGKVKGNFRLKELKNMKSGLPTTKSDNFPIPLVKQKGGQYTGFEISSHNDDFIIKIPFGRWQVKKEIDKYRPWEKFDFEQVRKSPKPISLLLSTQRRRRNKGWSKDEGTEAEIRKVMYGDYQTSYIEVKRGSKIGEKSAWMLNLSIDVPKIDKAADPSIIGGIDVGVKSPLVCAINNAFSRYSISDNDLFHFNKKVFARRRILLKKNRHRRAGHGAKNKLRPITILTEKSKRFRKKLIERWACEIADFFIKNKVGTVQMENLESMKRKEDSYFNIRLRGFWPYAEMQNKIEFKLKQYGIKIKKVAPNNTSRTCSECGHLNNYFSFEYRKKNKFPHFKCEKCNFKEDADYNAALNISNPKLKGTKEEL

SEQ ID NO: 2576 - protein, 726 aa, synthetic construct
SEVEFSHEYWMRRALTLAKRARDEREVPVGAVLVLNNRVIGVGWNRAVGLHDPTAHAEIMALRQGGLVMRNYRLIDATLYVTFEPCVMCAGAMIHSRIGRVVFGVRNSKHGAAGSLVNVLNYPGMNHRVEITEGILADECAALLCDFYRMPRQVFNARKKAQSSINPGGSSGGSSGSETPGTSESATPESSGGSSGSSAKNTITKTLKLRIVRPYNSAEVEKIVADEKNNREKIALEKNKDKVKEACSKHLKVAAYCTTQVERNACLFCKARRLDDKFYQKLRGQFPDAVFWQELGEILRQLQKQAAEIYNQSLIELYYEIFIKGRGFANASSVEHYLSDVCYTRAAELFKNAAIASGLRGKVKSNFRLKELKNMKSGLPTTKSDNFPIPLVKQKGGQYTGFEISSHNDDFIIKIPFGRWQVKKEIDKYRPWEKFDFEQVRKSPKPISLLLSTQRRKRNKGWSKDEGTEAEIRKVMSGDYQTSYIEVKRGSKTGEKSAWMLNLSIDVPKIDKGVDPSIIGGIDVGVKSPLVCAISNAFSRYSISDNDLFRFNKKMFARRRILLKKNRHKRAGHGAKNKLKPISILTGKSERFRKKLIERWACEIADFFIKNKVGTVQMENLESMKKKEDSYFNIRLRGFWPYAEMQNKIEFKLKQYGIEIRKVAPNNTSKTCSKCGHLNNYFNFEYRKRNKFPHFKCEKCNYKENADYNAALNISNPKLKSTKEEP

SEQ ID NO: 2577 - protein, 726 aa, synthetic construct
SEDEFSHEYWMRHALTLAKRARDGREVPVGAVLVLNNRVIGEGWNRAIGLHDPTAHAEIMALRQGGLVMQNYRLIDATLYVTFEPCVMCAGAMVHSRIGRVVFGVRNSKRGAAGSLMNVLDYPGMGHRVEITEGILADECAALLCDFYCMPRQVFNAQKRAQSSISSGGSSGGCSGSEMSGASESVTPKSSGGSSAGSTKNTITKTLKLRIVRPYNSAEVEKIVADEKNSREKIALERNKDKVKEACSEHLKVAAYCTTQVERNACLFCKARKLDDRFYQKLRGQFPDAVFWQETGEIFRQLQRQAAEIYNQSLIELYYEIFIKGKGFANASSVEHYLSDVCYTRAAELFRNAAIASGLRGKVKSNFRLKELKNMKSGLPTTKSDNFPIPLVKQKGGQYTGFEISSHNDDFIIKIPFGRWQVKKEIDKYRPWEKFDFEQVRKSPKPISLLLSTQRRKRNKGWSKDEGTEAEIRKVMNGDYQTSYIEVKRGSKIGEKSAWMLNLSIDVPKIDKGVDPSIIGGIDVGVKSPLVCAINNAFSRYSISDNDLFHFNKKMFARRRILLKKNGHKRAGHGAKNKLKPITTLTEKSGRFRKKLIERWACEIADFFIKNKVGTVQMENLESMKRKEDSYFNIRLRGFWPYAEMQNKIEFKLKQYGIEVRKVAPNNTSKTCSKCGHLNNYFNFEFRKKNKFPHFKCEKCNFKENADYNAALNISNPQLKSTKGEP

SEQ ID NO: 2578 - protein, 726 aa, synthetic construct
SEVEFSHEYWMRHALTLAKRARDEREVPVGAILVLNNRVIGVGWNRAIGLHDPTAHAEIMALRQGGLVMQNYRLIDATLYVTFEPCVMCAGAMIHSRIGRVVFGVRNSKHGAAGSLVNVLNYPGMNHRVEITEGILADECAALLCDFYRMPRQVFNARKEAQSSINSGGSSDGGSSSETPGTSESATPESSGGSPGGPAKNTITKTLRLRIVRPYNSTEVEKIVADEKNNREKIALEKNKDKVKEACSKHLKVAAYCTTQVERNACLFCKARKLDDKFYQKLRGQFPDAVFWQEVGEIFRQLQKQAAEIYNQSLIELYYEIFIKGKGFANASSVEHYLSDVCYSRAAELFKNAAVASGLRGKVKSNFRLKELKNMKSGLPTTKSDNFPIPLVKQKGGQYTGFEISNHNGDFIIKIPFGRWQAKKEIDKYRPWEKFDFEQVRKSPKPISLLLSTQRRKRNRGWSRDEGTEAEVKKVMNGDYQISYIEVKRGSKIGEKSAWTLNLSIDVPKIDKGVDPSIIGGIDVGVKSPLVCAISNALSRYSINDNDLFHFNKKMFARRRILLKKSKHKRAGHGAKNKLKPITILTEKSRRFRKKLIERWACEIADFFIKNKVGTVQMENLEGMKRKEDSYFNIRLRGFWPYAEMQNKIEFKLKQYGIEIRKVAPNNTSKTCSKCGHLNSYFNFEYRKKNKFPHFKCEKCNFRENADYNAALNISNPKLRSTKEEP

SEQ ID NO: 2579 - protein, 726 aa, synthetic construct
SEVEFSHEYWMRHALTLAKRARDEREVPVGAVLVLNNRVIGEGWNRAIGLHDPTAHAEIMALHQGGLVMQNYRLIDATLYVTFEPCVMCAGAMIHSRIGRVVFGARNSKRGAAGSLMNVLSYPGMNHRVEITEGVLADECAALLSDFYRMPRRVFDAQKRAQSSINSGGSSGGGSGSETPSTSESTTPESSGGSSGGPAKNTITKTLKLRIVRPYNSAEVEKIVADEKNNREKTALEKNKDKVKEACSKHLKVAAYCTTQVERNACLFCKARKLDDKFYQKLRGQFPDAVFWQELGEIFRQLQKQAAEIYNQSLIELYYEIFIKGKGFANASSVEHYLSDVCYTRAAELFKNAAIASGLRGKVKSNFRLKELKNMKSGLPTTKSDNFPIPLVKQKGGQYAGFEISSHNDDFIIKIPFGRWQVKKEIDKYRPWEKFDFEQVRKSPKPISLLLSTRRRKRNKGWSKDEGTEAEIRKVMNGDYQTSYIEVKRGSKIGEKSAWMLNLSIDVPKIDKGVDPSIIGGIDVGVKSPLVCAINNAFGRYSISDNDLFHFNKKMFARRRILLKKNRHKRAGHGAKNKLKPITILTEKSKRFRKKLIERWVCEVADFFIKNKVGTVQMENLESMKRKEDSYFNIRLRGFWPYAEMQNRIELKLKQYGIEVRRVAPNNTSRTCSKCGHLNNYFNFEYRKKNKFPHFKCEKCDFREDADYNAALNISNPKLKSTKEEP

SEQ ID NO: 2580 - protein, 726 aa, synthetic construct
SEVEFSHEYWMRHALTLAKRARDEREVPVGAVLVLNNRVIGVGWNRAIGLHDPTAHAEIMALRQGGLVTQNYRLIDATLYVTFEPCVMCAGAMIHSRIGRVVFGVRNSKHGAAGSLMDVLNYPGMNHRVEITEGILADECAALLCDFYRMPRQVFSARKKAQSSINPGGSSGGSSGSKTPGTSESATPESSGGSSGGSAKSTITKTLKLRIVRPYNSAEVEKIVADEKNNREKIALEKNKGKVKEACSKHLEVAAYCTTQVERNACLFCKARKLDDKFYQRLRGQFPDAVFWQELGEIFRQLQRQAAEIYNQSLIELYYEIFIKGKGFANASSVEHYLSDVCYTRAAELFKNAAIASGLRGKVKSNFRLKELKNMKSGLPTTKSDNFPIPLVKQKGGQYTGFEISSHNDDFIIKIPFGRWQVRKEIDKYRPWEKFSFEQVRKSPKPISLLLSTQRRKRNKGWSKDEGTEAEIRKVMNGDYQTSYIEVKRGSKIGEKSAWMLSLSIDVPKIDKGVDPSIIGGIDVGVKSPLVCAINNAFNRYSISDNNLFHFNKKMFARRRILLKKNRHKRAGHGAKNKLRPISILTEKSERFRKKLIERWACEIADFFIKNKVGTVQMENLESMKRKEDSYFNIRLRGLWPYAEMQNKIEFKLKQYGIKIRKVAPNNTSKTCSKCGHLNNYFNFEYRKKNKFPHFKCEKCSFKENADYNAALNISNPKLKSTKEEP

SEQ ID NO: 2581 - protein, 726 aa, synthetic construct
GEVEFSHEYWMRHALTLARRARDEREVPVGAVLVLNNRVIGEGWNRAIGLHDPTAHAEIMALRQGGLVMQNYRLTDATLYVTFEPCVMCAGAMIHSRIGRVVFGVRNSKRGAAGSLVNVLSYPGMNHCVEITEGILVDECAALLCDFYRMPRRVLNAQKKAQSSISSGGSSGGSSGSETLGTSESTTPESSGGSSGGPAKNTITKTLKLRIVRPYNSAEVEKIVADEKNNREKTALEKNKDKVKEACSEHLKVAAYCTTQVERSACLFCKARKLDDKFYQKLRGQFPDAVFWQEIGEIFRQLQKQAAEIYNQSLIELYYEIFIKGKGFANASSVEHYLSDVCYTRAAELFKNAAIASGLRGKVKSNFRLKELKNMKSGLPTTKSDNFPIPLVKQKGGQYTGFEISSHNDDFIIKIPFGRWQVKKEVDKYRPWEKFDLEQVRKSPKPISLLLSTQRRKRNKGWSKDEGTEAEIRKVMNGDYQTSYIEVKRGSKTGEKSAWMLNLSIDVPKIDKGVDPCIIGGIDVGVKSPLVCAINNAFSRYSTSDNDLFHFNKKMFARRRILLKKNGHKRAGHGAKNKLKPITIMTEKSKRFRKKLIERWACEIADFFIKNKVGTVQMENLESMKRKEDSYFNIRLRGFWPYAEMQNKIEFKLKQYGIVVRKVAPNNTSRTCSKCGHLNNYFNFEYRKKNKFPHFRCEKCNFKEDADYNAALNISNPKLKSTKEEP

SEQ ID NO: 2582 - protein, 726 aa, synthetic construct
SEVEFSHEYWMRHALTLAKRARDEREVPVGAVLVLNNRVIGEGWNRAIGLHDPTAHAEIMALRQGGLVMQNCRLIDATLYVTFEPCVMCAGAMVHSRIGRVVFGVRNSKRGAAGSLMNVLDYPGMDHRVEITEGILADECAALLCDFYRMPHQVFNAQKKAQSSINSGGSSGGSSGSVTPGPSESATPESSGGSSGSSAKNTITKTLQLMIVRPYNSAEVEKIVADEKNNREKIALEKNKDKVKEACSKHLKVASYCTTQVERNACLFCKARKLDDKFYQRLRGQFPDAVFWQELGEIFRQLQKQAAEIYNQSLIELYYEIFIKGKGFANASSVEHYLSDVCYTRAAELFKNAAIASGLRGKVKSNFRLKELKSMKSGLPTTKSDNFPIPLVKQKGGQYTGFEISSHNSDFIIKIPFGRWQVKEEIDKYRPWEKFDFEQVRKSPKPISLLLSTQRRKRNKGWSKDEGTEAEIRKVMNGDYQTSYIEVKRGSKTGEKSTWMLNLSIDVPKIDKGVDPSIIGGIDVGVKSPLVCAINNAFSRYSISDNDLFRFNKKMFARRRILLGKNRHKRAGHGVKNKLKPITILTERSGRFRKKLIERWACEIADFFVKNKVGTVQMENLESMKRKEDSYFNIRLRGFWPYAEMQNKIEFKLKQYGIKVRKVAPNNTSKTCSKCGHLNNYFNFEYRKKNKFPHFKCEKCNFKENADYNAALNISDPKLKSTKEEH

SEQ ID NO: 2583 - protein, 726 aa, synthetic construct
SEVEFSHEYWMRHALTLAKRARDEREVPVGAVLVLNNRAIGEGWNRTIGLHDPTAHAEIMALRQGGLVMQNYRLTDATLYVTFEPCVMCAGAMIHSRIGRVVFGVRNSKRGAAGSLMNVLNYPGMNHCVEITEGILVDECAALLCDFYRMPRQVLNAQKKAQSSISSGGSSGGSSGSETPGASGSVIPKSSGGSSAGSTKDTITKTLKLRIVRPYNSAEVEKVVADEKNNREKIAMEKNKDKVKEACSKHLKVASYCTTQVERNACLFCKARKLDDKFYQKLRGQFPDAVFWQELGGIFRQLQKQAAEIYNQSLIELYYEIFIKGKGITNASRVEHYLSDVCYTRAAELFKNAAIASGLRNKIKSNFRLKELRNMKSGLPTTKSDNFPIPLVKQKGGQYTGFEIGNHNSDFIIKIPFGRWQAKKEIDKYRPWEKFDFEQVRKSPKPISLLLSTQRRRRNKGWSKDEGTEAEIRKVMNGDYQTSYIEVKRGSKIGEKSAWMLSLSIDVPKIDKGVDPSIIGGIDVGVKSPLVCAINNAFCRYSISDNDLFHFNKKMFARRRILLKKSRHKRAGHGAKNKLKPISILTEKSKRFRKKLIERWACEIADFFIKNKVGTVQMENLESMKRKEDSYFNIRLRGFWPYAEMQNKIEFKLKQYGIEIRKVAPNNTSKTCSKCGHLNNYFNFEYRKKNKFPHFKCERCNFKENADYNAALNISNPKLKSTKEEP

SEQ ID NO: 2584 - protein, 726 aa, synthetic construct
SEDEFSHEYWMRHALTLAKRARDRREVPVGAVLVLNNRVIGEGWNRAIGLHDPTAHAEIMALRQGGLVMQNYRLIDATLYVTFEPCVMCAGAMIHSRIGRVVFGVRNSKHGAAGSLVNVLNYPGMNHRVEITEGILADECAALLCDFYRMPRQVFNARKKAQSSINSGGPSGGSSGSETPGTSESATPESSGGSSGGSAKNTITKTLQLRIVRPYNSAEVEKIVTDEKNNREKIALEKNKDKVKEACSKHLKMASYCTTQVERNACLFCKARKLDDKFYQKLRGQFPDAVFWQELGGIFRQLQKQAAEIYNQSLIELYYEIFIKGKGITNASRVEHYLSDVCYTRAAELFKNAAIASGLRSKVRSNFRLKELKNMKSGLPTTKSDNFPIPLVKQKGGQYTGFEISSHNDDFIIKIPFGRWQVKKEIDKYRPWEKFDFEQVRKSPKPISLLLSTQRRKRNKGWSKDEGTEAEIKKVMNGDYQTSYIEVKRGSKIGEKSAWMLNLSIDVPKIDRGVDPSIIGGIDVGVKSPLVCAINNASSRYSISDNDLFHFNKKMFARRRILLKKNRHKRAGHGAKNKLKPLTILTGKSKRFRKKLIERWACEIADFFTKNKVGTVQMENLESMKRRGDSYFNIRLRGLWPYAEMQNRIEFKLKQYGIEIRKVAPNNTSKTCSKCGHLNSYFNFEYRKKNKFPHFKCEKCNFKENADYNAALNISNPKLKSTKEEP

SEQ ID NO: 2585 - protein, 726 aa, synthetic construct
SEVEFSHEYWMRHALTLAKRARDEREVPVGAVLVLNNRVIGEGWNRAIGLHDPTAHAEIMALRQGGLVMQNYRLDDATLYVTFEPCVLCAGAMVHSRIGRVVFGVRNSKRGAAGSLMNVLNYPGMNHRVEITEGILADECAALLCDFYHMPRQVFSAQKKAQSSINSGGSSGGSSGSETPGTSESATPKSSGGSSGGSAKNTITKALKLRIVRPYNSAEVEKIVADEKNSREKIALERNKDKVKEACSEHLKVAAYCTTQVERNACLFCKARKLDDRFYQKLRGQFPDAVFWQETGEIFRQLQRQAAEIYNQSLIELYYEIFIKGKGFANASSVEHYLSDVCYTRAAELFKNAAIASGLRGKVKSNFRLKELKNMKSGLPTTKSDNFPIPLVKQKGGQYTGFEISSHNDDFIIKIPFGRWQVKKEIDKYRPWEKFDFEQVRKSPRPISLLLSTQRRKRNKGWSRDEGTEAEIRKVMNGDYQTSYIEVKRGSKIGEKSAWMLNLSIDVPKIDKGVDPSIIGGIDVGVKSPLVCAINNALSRYSISDNDLFHFNKKMFARRRILLRKNRHKRAGHGAKNKLKPITIMTEKSKRFRKKLIERWACEIANFFVKNKVGTVQMENLESMKRKEDSYFNIRLRGLWPYAEMQNKIEFKLKQYGIEVRKVAPNNTSKTCSKCGHLNNYFNFEYRKRNKFPHFKCEKCNFKENADYNAALNISNPKLKSTKEEP

SEQ ID NO: 2586 - protein, 726 aa, synthetic construct
SEVELSHEYWMRHALTLAKRARDEREVPVGAVLVLNNRVIGEGWNRAIGLHDPTAHAEIMALRQGGLAMRNYRLVDATLYVTFEPCVLCAGAMVHSRIGRVVFGVRNSKRGAAGSLMNVLNHPGMNHRVEITGGILADECAALLCDFYRMPRQVFNAQKKARSNINSGGSSGGSSGSETLGTSESATPESSGGSSGGSAKNTITKTLKLRIVRPYNSAEVEKIVADEKNNREKIALEKNKNKVKEACSEHLKVAAYCTTQVERNACLFCKARKLDDKFYQKLRGQFPDAVFWQEIGEIFRQLQKQAAEIYNQSLVELYYEIFIKGKGIANASSVEHYLSDVCYTRAAELFKNAAIASGLRNKIKSNFRLKELRNMKSGLPTTKSDNFPIPLVRQKGGQYTGFEISNHNSDFIIKIPFGRWQVKKEIDKYRPWEKFDFAQVRKSPKPISLLLSTQRRKRNKGWSNDEGTEAEIRKVMNGDYQTSYIEVKRGSKIGEKSAWMLSLSIDVPKIDKGVDPSIVGGIDVGVKSPLVCAINNALGRFSISDNDLFHFNKKMFARRRILLRKNRHKRAGHGAKSKLKPITILTEKGERFRKKLIERWACEIANFFIKNKVGTVQMENLESMKRKEDSYFNVRLRGFWPYAEMQNKIEFKLKQYGIEIRKVAPNNTSKTCSRCGHLNNYFNFEYRRKNKFPHFKCEKCNFKEDADYNAALNISNPKLKGTKEEP

SEQ ID NO: 2587 - protein, 726 aa, synthetic construct
SEVEFSHEYWMRHALTLAKRARDEREVPVGAVLVLNNRAIGEGWNRATGLHDPTAHAEIMALRQGGLVMQNYRLIDATLYVTFEPCVMCAGAMVHSRIGRVVFGVRNSKRGAAGSLMNVLDYPGMGHRVEITEGILADECAALLCDFYCMPRQVFNAQKRAQSSINSGGSSGGSSGSETPGTSESATPESSCGGSSGSAKNTITKTLQLRIVRPYNSAEVEKIVADEKNSREKIALEKNKDKVKEACSEHLKVAAYCTTQVERNACLFCKARKLDDRFYQKLRGQFPDAVFWQEIGEIFRQLQKQAAEIYNQSLIELYYEIFIKGKGITNASSVEHYLSDVCYTRAAELFKNAAIASGLRGKVKSNFRLKELKNMKSGLPTTKSDNFPIPLVKQKGGQYTGFEISSHNDDFIIKIPFGRWQVKKEIDRYRPWEKFDFEQVRKSPKPISLLLSTQRRKRNKGWSKDEGTEAEIRKVMNGDYQTSYIEVKRGSKIGEKSAWMLNLSIDVPKIDKGVDPSIIGGIDVGVKSPLVCAINNAFSRYSISDNDLFHFNKKMFARRRILQKKNRHKRAGHGAKNKLRPITILAEKSERFRKKLIEKWACEIADFFIKNKVGTVQMENLESMKRKEDSYFNIRLRGFWPYAEMQNKIEFKLKQYGIEIRKVAPNNTSKTCSKCGHLNNYFNFEYRKKNKFPHFKCEKCNFKENADYNAALNISNPKLKSTKEEP

SEQ ID NO: 2588 - protein, 726 aa, synthetic construct; identical to SEQ ID NO: 684

SEQ ID NO: 2589 - protein, 726 aa, synthetic construct
SEVEFSHEYWMRHALTLAKRARDEREVPVGAILVLNNRVIGEGWNRAIGLHDPTAHAEIMALRQGGLVMQNYRLIDATLYVTFEPCIMCAGAMIHSRIGRVVFGVRNSKRGAAGSLTNVLNYPGMNHRVEITEGILVDECAALLCDFYRMPRQVFNAQKKAQSTINSGGSSGGSSGSETPDTSESPTPESSGGSPGGSAKNTITKTLKLRIVRPYNSAEVEKIVADEKNNREKIALEENKDKVREACSEHLKVAAYCTTQVERNACLFCKARKLDDKFYQKLRGQFPDAVFWQEIGEIFRQLQKQAAEIYNQSLIELYYEIFIKGKGFANASSVEHYLSDVCYTRAAELFKNAAIASGLRGKVKSSFRLKELKNMRSGLPTTKSDNFPIPLVKQKGGQYTGFEVSSHNDDFIIKIPFGRWQVKKEIDKYRPWEKFDFEQVRKSPKPISLLLSTRRRKRNKGWSKDEGTEAEIRKVMNGDYRTSYIEVKRGSKIGEKSAWMLNLSIDVPKIDKGVDPSIIGGIDVGVKSPLVCAINNAFSRYSISDNELFHFNKKMFARRRILLKKNRHKRAGHGAKNKLKPISVLTEKSGRFRKKLIERWACEIADFFIKNKVGTVQIENLESMKRKEDSYFNIRLRGFWPYAEMQNKIEFKLKQYGIEIRKVAPNNTSKTCSKCGHLNSYFNFEYRKKNKFPHFKCEKCNFKENADYNAALNISNPKLKSTKEEP

SEQ ID NO: 2590 - protein, 726 aa, synthetic construct
SEVEFSHEYWMRHALILAKRARDEREVPVGAVLVLNNRVIGVGWNRTIGLHDPTAHAEIMALRQGGLVMRNYRLIDATLYVTFEPCAMCAGAMIHSRIGRVVFGVRNSKRGAAGSLMNVLNYPGMNHRVEITEGILVDECAALLCDFYRMPRRVFNARKKAQSSINPGGPSGGSSGSETPGTSESATPESSGGSSGGSAKNTITKTLKLRIVRPYNSAEVEKIVADEKSNREKIALEKNKDKVKEACSKHLKVASYCTTQVERNACLFCKARRLDDKFYQKLRGQFPDAVFWQEIGEIFRQLQKQAAEVYNQSLVELYYEILIKGKGIANASSVEHYLSDVCYTRAAELFKNAAIASGLRNKIKSNFRLKELRNMKSGLPTTKSDNFPIPLVRQKGGQYTGFEISNHDGDFIIKIPFGRWQVKKEINKHRPWEKFDFEQVRKSPKPISLLLSTQRRKRNKCWSKDEGTEAEIRKVMNGDYQTSYIEVKRGSKIGEKSAWMLNLSIDVPKIDKGVDPSIIGGIDVGVKSPLVCAINNAFSRYSISDNDLFRFNKKMFARRRILLRKNRHKRAGHGAKNKLKPISILTGKSERFRKKLIERWACEIADFFIKNKVGTVQMEDLESMKRREDSYFNIRLRGFWPYAEMQNKIEFKLKQYGIVVRKVAPNNTSKTCSKCGHLNNYFDFEYRKKNKFPHFKCEKCNFKEDADYNAALNISNPKLKSTKEEP

SEQ ID NO: 2591 - protein, 726 aa, synthetic construct
SEVEFSHEYWMRHALTLAKRARDEREVPVGAVLVLNNRVIGEGWNRTTGLHDPTAHAEIMALRQGGLVMQNYRLVDATLYVTFEPCVLCAGAMVHSRIGRVVFGVRNSKRGAAGSLMNVLDYPGMNHRVEITEGILADECAALLCDFYRMPRQVFNAQKKARPNINSGGSSGGRSGSETPGTSESATPESSGGGSSGSAKNTITKTLQLRIVRPYNSAEVEKIVADEKNNREKIALEKNKGKVKEACSKHLKVASYCTTQVERNACLFCKARKLDDKFYQKLRGQFPDAVFWQELGGIFRQLQKQAAEIYNQSLIELYYEIFIKGKGITNASRVEHYLSDVCYTRAAELFKNAAIASGLRGKVKGNFRLKELKNMKSGLPTTKSDNFPIPLVKQKGGQYTGFEISSHNDDFIIKIPFGRWQAKKEIDKYRPWEKFDFEQVRKSPKPISLLLSTQRRKRNKGWSKDEGTEAEIRKVMNGDYQTSYIEVKRGSKIGEKGAWMLNLSIDVPKIDKGVDPSIIGGIDVGVKSPLVCAINNAFSRYSISDNDLFHFNKKMFARRRILLKKNRPKRAGHGAKNKLKPISILTEKSKRFRKKLIERWACEIADFFIKNKVGTVQMENLESMKRKEDSYFNIRLRGFWPYAEMQNKIEFKLKQYGIEIRKVAPNNTSKTCSKCGHLNNYFNFEYRRKNKFPHFKCEKCNFKEDADYNAAQNISNPKLKSTKEEP

SEQ ID NO: 2592 - protein, 726 aa, synthetic construct
SEVEFSHEYWMRHALTLAKRARDEREVPVGAILVLNNRVIGEGWNRAIGLHDPTAHAEIMALRQGGLVMQNHRLVDATLYVTFEPCVMCAGAMIHSRIGRVVFGVRNSKRGAAGSLTNVLNYPGMNHRVEITEGILVDECAALLCDFYRMPRQVFNAQRKAQSTINSGGLSGGSSGSKTPGTSESPTPESSGGSPVGSAKNTITKTLKLRIVRPYNSAEVEKIVADEKNNREKIALEKNKDKVKEACSKHLKVAAYCTTQVERNACLFCKARKLDDKFYQKLRGQFPDAVFWQEVGEIFRQLQKQAAEIYNQSLIELYYEIFIKGKGITNASRVEHYLSDVCYTRAAELFKNAAIASGLRSKVRSNFRLKELKNMKSGLPTTKSDNFPIPLVKQKGGQYTGFEISSHNSDFIIKIPFGRWQEKEEIDKYRPWEKFDFEQVRRSPKPISLLLSTQRRKKNKGWSKDEGTEAEIRRVMNGDYQTSYIEVKRGSKIGGKSAWMLNLSIDVPKIDKGVDPSIIGGIDVGVKSPLVCAINNSFSRYSICDNDLFRFNKKMFARRRILLKKNRHKRAGHGAKNKLKPISILTEKSKRFRKKLIERWACEIADFFIKNKVGTVQMENLESMKRREDSYFNIRLRGFWPYAEMQNKIEFKLKQYGIEIRKVAPNNTSKTCSKCGHLNNYFNFEYRKMNKFPHFKCEKCNFKENADYNAALNISNPKLKSTKEEP

SEQ ID NO: 2593 - protein, 726 aa, synthetic construct
SEVEFSHEYWMRHALTLAKRARDEREVPVGAVLVLNNRVIGEGWNRAIGLQDPTAHAEIMALRQGGLVMQNYRLIDATLYVTFEPCAMCAGAMVHSRIGRVVFGVRNSKRGAAGSLMNVLTYPGMDHRVEITGGILADECAALLCDFYRMPRRVFNAQKKAQSSINSGGSSGGSSGSVTPGTSESATPESSGGSFGGSAKNTITKTLQLRIVRPYNSAEVEKIVADEKNSREKIALEKNKDKVKEACGKHLKVASYCTTQVERNACLFCKARKLDDKFYQKLRGQFPDAVFWQELGEIFRQLQKQAAEIYNQSLIELYYEIFIKGKGLANASSVEHYLSDVCYTRAAELFKNAAIASGLRGKVKSNFRLKELKNMRSGLPTTKSDNFPIPLVKQKGGQYAGFEISSRNDDFIIKIPFGRWQVKKEIDKYRPWEKFDFEQVRKSPKPISLLLSTQRRKRNRGWGKDEGTEAEIKRVMNGDYQTSYIEVKRGSKIGEKSAWMLNLSIDVPKIDKGVDPRIIGGIDVGVKSPLVCAINNAFSRYSVSDNDLFHFNKKVFARRRILLKKNRHKRAGHGTKNKLKPITILAEKSERFRKKLIEKWACEIADFFIKNKVGTVQMENLESMKRKEDSYFNIRLRGFWPYAEMQDKIEFKLKQYGIEIRKVAPNNTSKTCSKCGHLNNYFNFEYRKMNKFPHFKCEKCNFKENADYNAALNISNPKLKSTKEEP

SEQ ID NO: 2594 - protein, 726 aa, synthetic construct
SEVEFSHEYWMRHALTLAKRARDEREVPVGAILVLNNRVIGEGWNRAIGLHDPTAHAEIMALRQGGLVMQNYRLIDATLYVTFEPCVMCAGAMIHSRVGRVVFGVRNSKHGAAGSLMNVLNYPGMNHRVEITEGILADECAALLCDFYRMPRRVFNARKKTQSSIDPGGPSGGSSGSETPGTSKSATPESSGGSSGGSAKNTITKTLKLRIVRPYNSAEVEKIVADEKNNREKIALEKNKDKVKEACSKHLKVAAYCTTQVERNACLFCKARRLDDKFYQKLRGQFPDAVFWQEIGEIFRQLQKQAAEIYNQSLVELYYEIFIKGKGIANTSSVEHYLSDVCYTRAAELFKNAAIASGLRNKIKSNFRLKELRNMKSGLPTTKSDNFPIPLVRQKGGQYTGFEISNHNGDFIIKIPFGRWQVKKEISKHRPWEKFDFEQVRKSPKPISLLLSTQRRKRNKGWGKDEGTEAEIRKVMNGDYQTSYIEVKRGSKIGEKSAWMLSLSVDVPKIDKGVDPSIIGGIDVGVKSPLVCAINNALSRYSISDNDLFHFNKKMFARRRILLRNNRHKRAGHGARNKLKPITVLTEKSERFRKKLIERWACEIANFFIKNRVGTVQMENLESMKRKEDSYFNVRLRGFWPYAEMQNKIEFKLKQYGIEIRKVAPNNTSKTCSRCGHLNNYFNFEYRRKNKFPHFKCEKCNFKENADYNAALNISDPKLKSTKEEP

SEQ ID NO: 2595 - protein, 726 aa, synthetic construct
SEVEFSHEYWMRHALTLAKRARDEREVPVGAVLVLNNRVIGEGWNRAIGLHDPTAHAEIMALRQGGLVMQNYRLSDATLYVTFEPCVMCAGAMILSRIGRVVFGVRNSKRGAAGSLMNVLNYPGMNHRVEITEGVLADECAALLCDFYRMPRQVLNAQKKAQSSINSGGSSGGGSGGETPGTSESATPESSGGSSGGSAKNTITKTLQLRIVRPYNSAEVEKIVADEKNNREKIALEKNKDKVKEACSKHLKVASYCTTQVERNACLFCKARKLDDKFYQKLRGQFPDAVFWQELGEIFRQLQKQAAEIYNQSLIELYYEIFIKGKGFANASSVEHYLSDVCYTRAAELFKNAAIASGLRGKVKSNFRLKELKNMKSGLPTTKSDNFPIPLVKQKGGQYTGFEISSHNDDLIVKIPFGRWQVKKEIDKYRPWEKFDFEQVRKSPKPISLLLSTQRRKRNKGWSKDEGTEAEIRKVMNGDYQTSYIEVKRGSKIGEKDAWMLNLSIDVPKIDKGVDPSIIGGIDVGVKSPLVCAINNAFSRYSISDNELFHFNKKMFARRRILLKKSRHKRAGHGAKNKLKPITILTEKSRRFRKKLIERWACEIADFFIKNKVGTVQMENLESMKRKEDSYFNIRLRGFWPYAEMQNKIEFKLKQYGIVIRKVAPNNTSRTCSKCGHLNNYFNFEYRKKNKFPHFKCEKCNFKENADYNAALNISNPKLKSTKEEP

SEQ ID NO: 2596 - protein, 726 aa, synthetic construct
SEVEFSHEYWMRHALTLAKRARDEREVPVGAILVLNNRVIGEGWNRAIGLHDPTAHAEIMALRQGGLVMQNYRLIDATLYVTFEPCVMCAGAMIHSRIGRVVFGVRNNKHGAAGSLVNVLNYPGMNHRVEITEGILADECAALLCDFYRMPRQVFNARKKAQSSTNPGGSSGGSSGSETPGTSESATPKSSGGSSGGSAKNTITKALKLRIVRPYNSAEVEKIVADEKNNRERIALEKNKDKVKEACSKHLKVAAYCTTQVERNACLFCKARKLDDKFYQKLRDQFPDAVFWQEIGEIFRQLQKQAAEAYNQSLVELYYEIFIKGKGIANASNVEHYLSDVCYTRAAELFKNAAIASGLRGKVKSNFRLRELKNMKSGLPTTKSDNFPIPLVKQKGGQYTGFEISNHNSDFIIKIPFGRWQVKKEINKYRPWEKFDFEQVRKSPKPISLLLSTQRRKRNKGWSKDEGTEAEIRKVMNGDYQTSYIEVKRGSRIGEKSAWMLSLSIDVPKIDRGVDPSVIGGIDVGVKSPLVCAINNALSRYSISDNDLFHFNKKMFARRRILLKKNRHRRAGHGARNKLKPITVLTEKSKRFRKKLIERWACEIANFFVKNKVGTVQMENLESMKRKEDSYFNIRLRGLWPYAEMQNKIEFKLKQYGIEVRKVAPNNTSKTCSKCGHLNNYFNFEYRKRNKFPHFKCEKCNFKENADYNAALNISNPKLKGTKEEP

SEQ ID NO: 2597 - protein, 726 aa, synthetic construct
SEVEFSHEYWMRHALTLARRARDEREVPVGAVLVLNNRVIGEGWNRAIGLHDPTAHAEIMALRQGGLVMQNYRLVDATLYVTFEPCVLCAGAMVHSRIGRVVFGVRNSKRGAAGSLMNVLNYPGMNHRVEITEGILADECAALLCDFYRMPRQVFNARKKARSNINSSGSSGGSSGSETPGTSESATPESSGGSSGGSAKNTITKTLKLRIVRPYNSAEVEKIVADEKNNREKIALEKNKDKVKEACSEHLKVAAYCTTQVERNACLFCRARKLDDKFYQKLRGQFPDAVFWQEIGEIFRQLQKQAAEIYNQSLIELYYEIFIKGKGFANASSVEHYLSDVCYTRAAELFKNAAIASGLRGKVKSNLRLKELKNMKSGLPTTKSDNFPIPLVKQKGGQYTGFEISSHNDDFIIKIPFGRWQVKKEIDKYRPWEKFDFEQVRKSPKPISLLLSTQRRKRNKGWGKDEGTEAEIRKVMNGDYQTSYIEVKRGSKIGEKSAWMLSLSIDVPKIDKGVDPRIIGGIDVGVKSPLVCAINNAFSRYSISDNDLFHFNKKMFARRRILLKKNRHKRAGHGAKNKLKPITILTERSVRFRKKLIERWACEIADFFIKNKVGTVQMENLESMKGKEDSYFNIRLRGFWPYAEMQNKIEFKLKQYGIEIRKVAPNNTSKTCSKCGHLNNYFNFEYRKKNKFPYFKCEKCNFEENADYNAALNISNPQLKSTKGEP

SEQ ID NO: 2598 - protein, 726 aa, synthetic construct
SEDEFSHEYWMRHALTLAKRARDGREVPVGAVLVLNNRVIGEGWNRAIGLHDPTAHAEIMALRQGGLVMQNYRLTDATLYVTFEPCVLCAGAMVHSRIGRVVFGARNSKRGAAGSLMNILNYPGMNHRVEITEGILADECAALLCDFYRMPRQVFNAQKKAQSSINSGGSSGGSSGSETPGTSESATPESSGGSSGGSAKNTITKTLKLRIVRPYNSAEVEKIVADEKNSREKIALERNKDKVKEACSRHLKVAAYCTTQVERNACLFCKARKLDDKFYQKLRGQFPDAVFWQELGEIFRQLQKQAAEIYNQSLIELYYEIFIKGKGFANASSVEHYLSDVCYTRAAELFKNAAIASGLRGKVKSNFRLKELKNMKSGLPTTKSDNFPIPLVKQKGGQYTGFEISSHNSDFIIKIPFGRWQEKEEIDKYRPWEKFDFEQVRRSPKPISLLLSTQRRKKNKGWSKDEGTEAEIRRVMNGDYQTSYIEVKRGSKIGEKSAWMLNLSIDVPKIDKGVDPSIIGGIDVGVKSPLVCAINNAFSRYSISDNDLFHFNKKMFARRRILLRKNRHKRAGHGARNKLKPITVLTEKSERFRKKLIERWACEIANFFIKNKVGTVQMENLESMKRKEDSYFNIRLRGFWPYAEMQNKIEFKLKQYGIEIRKVAPNNTSKTCSKCGHLNNYFNFEYRKKNKFPHFKCEKCNFKENADYNAALNISNPKLKSTKEEP

SEQ ID NO: 2599 - protein, 726 aa, synthetic construct
SEVEFSHEYWMRHALTLAKRARDEREVPVGAVLVLNNRVIGEGWNRAIGLHDPTAHAEIMALRQGGLVMQNYRLIDATLYVTFEPCVMCAGAMVHSRIGRVVFGVRNSKRGAAGSLMNVLDYPGMGHRVEITEGILADECAALLCDYYRMPRQVFNARKKAQSSINSGGSSDGGSGSETPGTSESATPESSGGSSGGSAKNTITKTLKLRIVRPYNSAEVEKIVADEKNNREKIALEKNKDKVKEACSKHLKVAAYCTTQVERNACLFCKARRLDDKFYQKLRGQFPDAVFWQEIGEIFRQLQKQAAEIYNQSLIELYYEIFIKGKGFANASSVEHYLSDVCYTRAAELFKNAAIAGGLRGKVKSNFRLKELKSMKSGLPTTKSDNFPIPLVKQKGGQYTGFEISSHNDDFIIKIPFGRWQEKKEIDKYRPWEKFGFEQVRKSPKPISLLLSTQRRKRNKGWSKDEGTEAEIRKVMNGDYQTSYIEVKRGSKIGEKSAWMLSLSIDVPKVDKGVDHSIVGGIDVGVKSPLVCAINNAFSRYSISDNDLFHFNKKMFARRRILLKKTRHKRAGHGAKNKLKPITIMTEKSKRFRKKLIERWACEIADFFIKNKVGTVQMENLESMKRREDNYFNIRLRGFWPYAEMQNKIEFKLKQYGIVVRKVAPNNTSKTCSKCGHLNNYFNFEYRKKNKFPHFKCEKCNFKEDADYNAALNISNPKLKSTKGEP

SEQ ID NO: 2600 - protein, 726 aa, synthetic construct
SEVEFSHEYWMRHALTLAKRARDEREVPVGAVLVLNNRVIGEGWNRAIGLHDPTAHAEIMALRQGGLAMRNYRLVDATLYVTFEPCVLCAGAMVHSRIGRVVFGVRNSKRGAAGSLMNVLNHPGMNHRVEITGGILADECAALLCDFYRMPRQVFNAQKKARSNINSGGSSGGSSGSETLGTSESATPESSGGSSGGSAKNTITKTLKLRIVRPYNSAEVEKIVADEKNNREKIALEKNKDKVREACSKHLKVASYCTTQVERNACPFCKARKLDDKFYQKLRGQFPDAVFWQELGEILRQLQKQAAKIYNQSLIELYYEIFIKGKGFANASSVEHYLSDVCYTRAAELFRNAAIASGLRGKVKGNFRLKELKSMKSGLPTTKSDNFPIPLVKQKGGQYTGFEISSHNDDFIIKIPFGRWQVKKEINKFRPWEKFDFEQVRKSPKPISLLLSTQRRKRNKGWSKDEGTEAEIRKVMNGDYRTSYIEVKRGSKIGEKGAWMLNLSIDVPKIDKGVDPSIIGGIDVGVKSPLVCAINNALSRYSISDNDLFHFNKKMFARRRILLRKNRHKRAGHGARNKLKPITVLTEKSERFRKKLIERWACEIANFFIKNKVGTVQMENLESMKRREDSYFNIRLRGFWPYAEMQNKIEFKLKQYGIEIRKVAPNNTSKTCSKCGHLNNYFNFEFRKKNKFPHFKCEKCNFKENADYNAALNISNPKLKSTKEEP

SEQ ID NO: 2601 - protein, 726 aa, synthetic construct
SEDEFSHEYWMRHALTLAKRARDGREVPVGAVLVLNNRVIGEGWNRAIGLHDPTAHAEIMALRQGGLVMQNYRLIDATLYVTFEPCVMCAGAMVHSRIGRVVFGVRNSKRGAAGSLMNVLDYPGMGHRVEITEGILADECAALLCDFYRMPRQVFNAQKRAQSSINSGGSSGGSSGSETPGTSESATPESSGGGSSGSAKNTITKTLQLRIVRPYNSAEVEKIVADEKNNREKIALEKNKGKVKEACSKHLEVASYCTTQVERNACLFCKARKLDDKFYQKLRGQFPDAVFWQELGEVFRQLQKQAAEIYNQSLIELYYEIFIKGKGLTNASSVEHYLSDVCYTRAAELFKNAAIASGLRGKVKSNFKLKELKSMKSGLPSTKSDNFPIPLVKQKGGQYTGFEIRGHNDDLIIKIPFGRWQVKKEIDKYRPWEKFDFEQVRKSPKPISLLLSTQRRKRNKGWSKDEGTEAEIRKVMNGDYQTSYIEVKRGSKIGEKSAWMLNLSIDVPKIDKGVDPSIIGGIDVGVKSPLVCAINNAFSRYSISDNDLFHFNKKMFARRRILLKKNGHKRAGHGAKNKLKPISILTEKSKRFRKKLIERWACEIADFFIKNKVGTVQMENLESMKGKEDSYFNIRLRGFWPYAEMQNKIEFKLKQYGIEIRKVAPNNTSKTCSRCGHLNNYFNFEYRKMNKFPHFKCEKCNFKENADYNAALNISNPKLKSTKEEP

SEQ ID NO: 2602 - protein, 726 aa, synthetic construct
SEVEFSHEYWMRHALTLAKRARDEREVPVGAVLVLNNRVIGEGWNRAIGLHDPTAHAEIMALRQGGLVMQNYRLIDATLYVTFEPCVMCAGAMVHSRIGRVVFGVRNSKRGAAGSLMNVLDYPDMGHRVEITEGILADECAALLCDFYCMPRQVFNAQKRAQSSINSGGSSGGSSGSETPGTSESATPESSGGGSSGSAKNTITKTLKLRIVRPYNSAEVEKIVADEKNNRERIALEKNKDKVKEACSKHLKVAAYCTTQVERNACLFCKARKLDDKFYQKLRGQFPDAVFWQETGEIFRQLQRQAAEIYNQSLIELYYEIFIKGKGFANASSVEHYLSDVCYTRAAELFRNAAIASGLRGKVKGNFRLKELKNMKSGLPTTKSDNFPIPLVKQKGGQYTGFEISSHNDDFIIKIPFGRWQVKKEIDKYRPWEKFDFEQVRKSPKPISLLLSTQRRKRNKGWSKDEGTEAEIRKVMNGDYQTSYIEVKRGSKTGEKSAWMLNLSIDVPKIDKGVDPSIIGGIDVGVKSPLVCAISNAFSRYSISDNDLFHFNKKMFARRRILLKKSKHKRAGHGAKNKLKPITILTEKSRRFRKKLIERWACEIADFFIKNKVGTVQMENLESMKRREDSYFNIRLRGFWPYAEMQNRIELKLKQYGIEIRRVAPNNTSRTCSKCGHLNNYFNFEYRKKNKFPHFKCEKCNFREDADYNAALNISNPKLKSTKEKP

SEQ ID NO: 2603 - protein, 726 aa, synthetic construct
SEVEFSHEYWMRHALTLAKRARDEREVPVGAILVLNNRVIGEGWNRAIGLHDPTAHAEIMALRQGGLVMQNYRLIDATLYVTFEPCVMCAGAMIHSRIGRVVFGVRNNKHGAAGSLVNVLNYPGMNHRVEITEGILADECAALLCDFYRMPRQVFNARKKARSSINLGGSSGGSSGSETPGTSESATPESSSGSSGGSAKNTITKALKLRIVRPYNSAEVEKIVADEKNNREKIALEKNKDKVEEACSRHLKVATYCTTQVERNACLFCKARKLDDKFYQKLRGQFPDAVFWQEIGEIFRQLQKQAAEIYNQSLIELYYEIFIEGKGSANARSVEHYLSDVCYTRAAELFKNAAIASGLRGKVKGNFRLKELKSMKSGLPTTKSDNFPIPLVKQKGGQYTGFEISSHNDDFIIKIPFGRWQVKKEIDKYRPWEKFDFEQVRKSPKPISLLLSTQRRKRNKGWSKDEGTEAEIRKVMNGDYQTSYIEVKRGSKTGEKSAWMLNLSIDVPKIDKGVDPSIIGGIDVGVKSPLVCAINDAFSRYSISDNDLFRFNKKMFARRRILLKKNRHKRAGHGTKNKLKPITILTEKSGRFRKKLIERWACEIADFFIKNKVGTVQMENLESMKRKEDSYFNIRLRGFWPYAEMQNKIEFKLKQYGIEIRKVAPNNTSKTCSKCGHLNNYFDFEYRKKNKFPHFKCEKCNFKENADYNAALNISNPKLKSTKEEP

SEQ ID NO: 2604 - protein, 726 aa, synthetic construct
SEVEFSHEYWMRHALTLAKRARDEREVPVGAVLVLNNRVIGEGWNRAIGLHDPTAHAEIMALRQGALVMQNYRLTDATLYVTFEPCVMCAGAMVHSRIGRVVFGVRNSKRGAAGSLMNVLNYPGVNHCVEITEGILVDECAALLCDFYRMPRQVLNAQKKAQSSISSGGSSGGCSGGEMSGASESVTPKSSGGSSAGSTKNTITKTLKLRIVRPYNSAEVEKIVADEKNSREKIALERNKDKVKEACSEHLKVAAYCTTQVERNACLFCKARKLDDRFYQKLRGQFPDAVFWQETGEIFRQLQRQAAEIYNQSLIELYYEIFIKGKGFANASSVEHYLSDVCYTRAAELFKNAAIASGLRGKVKSNFRLKELKSMKSGLPTTKSDNFPIPLVKQKGGQYTGFEISSHNSDFIIKIPFGRWQVKEEIDKYRPWEKFDFEQVRKSPKPISLLLSTQRRKRNKGWSKDEGTEAEIRKVMNGDYQTSYIEVKRGSRIGEKSAWMLNLSIDVPKIDKGVDPSIIGGIDVGVKSPLVCAINNALSRYSISDNDLFHFNKKMFARRRILLRKNRHKRAGHGAKNKLKPITIMTEKSKRFRKKLIERWACEIADFFIKNKVGTVQMENLESMKRKEDSYFNIRLRGFWPYAEMQNKIEFKLKQYGIKIRKVAPNNTSKTCSKCGHLNNYFSFEYRKKNKFPHFKCEKCNFKENADYNAALNISNPKLMSTKEEP

SEQ ID NO: 2605 - protein, 726 aa, synthetic construct
SEVEFSHEYWMRHALTLAKRARDEREVPVGAILVLNNRVIGEGWNRAIGLHDPTAHAEIMALRQGGLVMQNYRLIDATLYVTFEPCVMCAGAMIHSRVGRVVFGIRNSKRGAAGSLMNVLNYPGMNHRVEITEGILVDECAALLCDFYRMPCQVLNAQKKARSNINSGGSSGGSSSSETPGTSGSATPEGSGGSSGGSAKNTITKTLKLRIVRPYNSAEVEKIVADEKNNREKIALEKNKDKVKEACSKHLKVASYCTTQVERNACPFCKARKLDDKFYQKLRGQFPDAVFWQELGEIFRQLQKQAAEVYNQSLIELYYEIFIKGKGFANASSVEHYLSDVCYTRAAELFKNAAIASGLRGKVKSNFRLKELKNMKSGLPTTKSDNFPIPLVRQKGGQYTGFEISNHNSDFIIKIPFGRWQVKKEIDKYRPWEKFDFAQVRKSPKPISLLLSTQRRKRNRGWSKDESTEAEIRKVMNGDYQTSYIEVKRGSKIGEKSAWMLNLSIDVPKIDKGVDPSIIGGIDVGVKSPLVCAINNAFSRYSISDNDLFHFNKKMFARRRILLKKSKHKRAGHGAKNKLKPITILTEKSKRFRKKLIERWACEIADFFIKNKVGTVQMENLESMKKKEDSYFNIRLRGFWPYAEMQNKIEFKLKQYGIEIRKVAPNNTSRTCSKCGHLNNYFNFEYRKKNKFPHFKCEKCNFKEDADYNAALNISNPKLKSTKEEP

SEQ ID NO: 2606 - protein, 726 aa, synthetic construct
SEVEFSHEYWMRHALTLAKRARDEREVPVGAVLVLNNRVIGEGWNRAVGLHDPTAHAEIMALRQGGLVMQNYRLTDATLYVTFEPCVMCAGAMIHSRIGRVVFGVRNSKRGAAGSLMNVLNYPGMNHCVEITEGILVDECAALLCDFYRMPRQVLNAQKKAQSSISSGGSSGGSSCSETPGASESVTPKSSGGSSAGSTKNTITKTLQLRIVRPYNSAEVEKIVADEKNNREKIALEKNKDKVKEACSKHLKVASYCTTQVERNACPFCKARKLDDKFYQKLRGQFPDAVFWQELGEILRQLQKQAAEIYNQSLIELYYEIFIKGRGFANASSVEHYLSDVCYTRAAELFKNAAIASGLRGKVKSNFRLKELKNMKSGLPTTKSDNFPIPLVKQKGGQYTGFEISSHNDDFIIKIPFGRWQAKEEINKYRPWEKFDFEQVRKSPKPISLLLSTQRRKKNKGWSKDEGTEAEIRRVMNGDYQTSYIEVKRGSKIGEKSAWMLNLSIDVPKIDKGVDPSIVGGIDVGVKSPLVCAINNAFSRYSISDNELFHFNKKMFARRRILLKKNWHKRAGHGAKNKLKPISILTEKSERFRKKLIERWACEIANFFIKNKVGTVQMENLEGMKRKEDSYFNIRLRGFWPYAEMQNKIEFKLKQYGIEIRKVAPNNTSKTCSKCGHLNNYFNFGYRKKNKFPHFKCEKCNFKENADYNAALNISNPKLKSTKGEP

SEQ ID NO: 2607 - protein, 726 aa, synthetic construct; identical to SEQ ID NO: 2544

SEQ ID NO: 2608 - protein, 726 aa, synthetic construct
NEVEFSHEYWMRHALTLAKRARDEREVPVGAVLVLNNRVIGEGWNRAIGLHDPTAHAEIMALRQGGLVMQNYRLVDATLYVTFEPCVLCAGAMVHSRIGRVVFGVRNSKRGAAGSLMNVLNYPGMNHRVEITEGILADECAALLCDFYRMPRQVLNAQKKAQSSISSGGSSGGCSGSEMPGASESVTPKSSGGGSAGSTKNTITKTLKLRIVRPYNSAEVEKIVADEKNSREKIALERNKDKVKEACSEHLKVAAYCTTQVERNACLFCKARKLDDRFYQKLRGQFPDAVFWQETGEIFRQLQRQAAEIYNQSLIELYYEIFIKGKGFANASSVEHYLSDVCYTRAAELFKNAAIASGLRGKVKSNFRLKELKNMKSGLPTTKSDNFPIPLVKQKGGQYTGFEISSHNDDFIIKIPFGRWQVKKEIDKYRPWEKFDFERVRKSPKPISLLLSTQRRKRNKGWGKDEGTEAEIRKVMNGDYQTSYIEVKRGSKTGEKSAWMLNLSIDVPKIDKGVDPSIIGGIDVGVKSPLVCAINNAFSRYSISDNDLFRFNKKMFARRRILLKKNRHKRAGHGAKNKLKPISILTGKSERFRKKLIERWACEIADFFIKNKVGTVQMENLESMKRREDSYFNIRLRGFWPYAEMQSKIEFKLKQYGIKIRKVAPNNTSKTCSKCGHLNNYFSFEYRKKNKFPHFKCEKCNFKENADYNAALNISNPKLKSTKEEP

SEQ ID NO: 2609 - protein, 726 aa, synthetic construct; identical to SEQ ID NO: 684

SEQ ID NO: 2610 - protein, 726 aa, synthetic construct
SEVEFSHEYWMRHALTLAKRARDEREVPVGAILVLNNRVIGEGWNRAIGLHDPTAHAEIMALRQGGLVMQNYRLIDATLYVTFEPCVMCAGAMIHSRIGRVVFGVRNNKHGAAGSLVNVLNYPGMNHRVEITEGILADECAALMCDFYRMPRQVFNARKKAQSSINPGGSSGGSSGSETPGTSESATPESSGGSSGGSAKNTITKTLKLRIVRPYNSAEVEKIVADEKNNREKIALEKNKDKVKEACSEHLKVAAYCTTQVERSACLFCKARKLDDKFYQRLRGRFPDAVFWQEIGEIFRQLQKQAAEIYNQSLIELYYEIFIKGKGFANASSVEHYLSDVCYTRAAELFKNAAIASGLRGKVKSNFRLKELKSMKSGLPTTKSDNFPIPLVKQKGGQYTGFEISSHNDDFIIKIPFGRWQVKKEIDKYRPWERFDFEQVRKSPKPISLLLSTQRRKRNKGWSKDEGTEAEIRRVMNGNYQTSYIEVKRGSKIGEKSAWMLNLSIDVPKIDKGVDPSIIGGIDVGVKSPLVCAINNSLSRYSICDNDLFRFNKKMFARRRILLKKNRHKRAGHGAKNKLKPITILTKKSERFRKKLIERWACEVADFFIKNKVGTVQMENLESMKRKEDSYFNIRLRGFWPYAEMQNKIEFKLRQYGIEIRKVAPNNTSKTCSKCGHLNNYFDFEYRRKNKFPLFKCEKCSFKENADYNAALNISSPKLKSTKGEP

SEQ ID NO: 2611 - protein, 726 aa, synthetic construct
SEVEFSHEYWMRHALTLAKRARDEREVPVGAILVLNNRVIGEGWNRAIGLHDPTAHAEIMALRQGGLVMQNYRLTDATLYVTFEPCVMCAGAMIHSRIGRVVFGVRNSKRGAAGSLMNVLNYPGMNHRVEITEGILADECAGLLCDFYRMPRQVFSARKKAQSSINPGGSSGGSSGGKAPGTSESATLESSGGSSGDSAKNSITKTLKLRIVRPYNSAEVEKIVADEKNNREKIALEKNKGKVEEACSKHLKVATYCTTQVERNACLFCKARKLDDKFYQKLRGQFPDAVFWQEIGEIFRQLQKQAAEIYNQSLIELYYEIFIEGKGSANARSVEHYLSDVCYTRAAELFKNAAIASGLRGKVKGNFRLKELKSMKSGLPTTKSDNFPIPLVKQKGGQYTGFEISSHNDDFIIKIPFGRWQVKEEIDKYRPWEKFDFEQVRKSPKPISLLLSTQRRKKNKGWSKDEGTEAEIRKVMNGDYQTSYIEVKRGSRIGEKSAWMLNLSIDVPKIDKGVDPSIIGGIDVGVKSPLVCAINNALSRYSISDNDLFHFNKKMFARRRILLRKNRHKRAGHGAKNKLKPITIMTEKSKRFRKKLIERWACEIADFFIKNKVGTVQMENLESMKRKEDSYFNIRLRGFWPYAEMQNKIEFKLKQYGIVVRKVAPNNTSKTCSKCGHLNNYFNFEYRKKNKFPHFKCEKCNFKENADYNAALNISNPRLKSTKEEP

SEQ ID NO: 2612 - protein, 726 aa, synthetic construct
SEVEFSHEYWMRHALTLAKRARDEREVPVGAVLVLNNRVIGVGWNRAVGLHDPTAHAEIMALRQGGLVMQNYRLIEATLYVTFEPCIMCAGAMIHSRIGRVVFGVRNSKRGAAGSLMNVLNYPGMNHRVEITEGILADECAALLCDYYRMPRQVFNARKKAQSSINSGGSSDGGSGSETPGTSESATPESSGGSSGSSAKNTITKTLKLRIVRPYNSAEVEKIVADEKNNREKIALEKNKDKVKEACSKHLKVAAYCTTQVERNACLFCKARKLDDKFYQKLRGQFSDAVFWQEIGEIFRQLQKQAAEIYNQSLVELYYEILIKGKGFANASSVEHYLSDVCYTRAAELFKNAAIASGLRNKIKSNFRLKELRNMKSGLPTTKSDNFPIPLVRQKGGQYTGFEISNHDGDFIIKIPFGRWQVKKEINKHRPWEKFDFEQVRKSPKPISLLLSTQRRKRNKGWSKDEGTEAEIRKVMNGDYQTSYIEVKRGSKTGEKSAWMLSLSIDVPKIDKGVDPSIIGGIDVGVKSPLVCAINNAFSRYSISDNDLFRFNKKMFARRRILLKKNRHKRAGHGAKNKLKPISILTGKSERFRKKLIERWACEIADFFVKNKVGTVQMENLESMKRKEDSYFNIKLRGFWPYAEMQNKIEFKLKQYGIKVRRVAPNNTSKTCSKCGHLNNYFSFEYRKKNKFPHFKCEKCNFKENADYNAALNISNPKLKSAKEEP

SEQ ID NO: 2613 - protein, 726 aa, synthetic construct
SEVEFSHEYWMRHALTLAKRARDEREVPVGAVLVLSNRVIGEGWNRAIGLHDPTAHAEIMALRQGGLVMQNYRLIDATLYVTFEPCVMCAGAMVHSRIGRVVFGVRNSKRGAAGSLMNVLDYPGMGHRVEITEGILADECAALLCDFYCMPRQVFNAQKRAQSSINSGGSSGGSSGSETPGTSESATPESSGGGSSGSAKNTITKTLQLRIVRPYNSAEVEKIVADEKNSREKIALEKNKDKVKEACSKHLKVASYCTTQVERNACPFCKARKLDDKFYQKLRGQFPDAVFWQELGEILRQLQKQAAEIYNQSLIELYYEIFIKGRGFANASSVEHYLSDVCYTRAAELFKNAAIASGLRNKIKSNFRLKELRNMKSGLPTTKSDNFPIPLVRQKGGQYTGFEISNHNGDFIIKIPFGRWQVKKEINKHRPWEKFDFEQVRKSPKPISLLLSTQRRKRSKGWSKDEGTEAEIRKVMNGDYQTSYIEVKRGSKIGEKSAWMLNLSIDVPKIDKGVDPSITGGIDVGVKSPLVCAINNALSRYSISDNDLFHFNKKMFARRRILLKRNGHKRAGHGAKNKLKPVSILTEKSERFRKKLIERWACEIADFFIKNKVGTVQMENLESMKRKEDSYFNIRLRGFWPYAEMQNKIEFKLKQYGIEIRKVAPNNTSKTCSKCGHLNNYFNFEYRKKNKFPHFKCEKCNFKENADYNAALNISNPKLKSTKEEP

SEQ ID NO: 2614 - protein, 726 aa, synthetic construct
SEVEFSHEYWMRHALTLARRARDEREVPVGAVLVLNNRVIGEGWNRAIGLHDPTAHAEIMALRQGGLVMQNYRLIDATLYVTFEPCVMCAGAMIHSRIGRVVFGVRNSKHGAAGSLVNVLNYPSMNHRVEITEGILADECAALLCDFYRMPRQVFNARKKTQSSINPGGSSGGSSGSETPGTSESATPGSSSGSSGGSAKNTITKTLKLRIVRPYNSAEVEKIVAEEKDNREKIALEKNKDKVREACSKHLKVAAYCTTQVERNACLFCKARKLDDKFYQKLRGQFPDAVFWQEIGEIFRQLQKQAAEIYNQSLIELYYEIFIKGKGFANASSVEHYLSDVCYTRAAELFKNAAIASGLRGKVKSNFRLKELKNMKSGLPTTKSDNFPIPLVKQKGGQYTGFEISSHNGDFIIKIPFGRWQVKKEINKHRPWEKFDFEQVRKSPKPISLLLSTQRRKRNKGWSKDEGTEAEIRKVMNGDYQTSYIEVKRGSKIGEKSAWMLNLSIDVPKIDKGVDPSIIGGIDVGVKSPLVCAINNAFSRYSISDNDLFHFNKKMFARRRILLRKNRHKRAGHGTKNKLKPITILTEKSGRFRKKLIERWACEIANFFIKNKVGTVQMENLESMKRRGDSYFNIRLRGFWPYAEMQNKIEFKLKQYGIKIRKVAPNNTSKTCSKCGHLNNYFSFEYRKKNKFPHFKCEKCNFKEDADYNAALNISNPKLKSTKEEP

SEQ ID NO: 2615 - protein, 726 aa, synthetic construct
SEDEFSHEYWMRHALTLAKRARDGREVPVGAVLVLNNRVIGEGWNRAIGLHDPTAHAEIMALRQGGLVMQNYRLIDATLYVTFEPCVMCAGAMVHSRIGRVVFGVRNSKRGAAGSLMNVLDYPGMGHRVEITEGILADECAALLCDFYCMPRQVFNAQKKARSNINSGGSSGGSSGSETPGTSESATPESSGGSSGGSAKNTITKTLKLRIVRPYNSAEVEKIVADEKNNREKIALEKNKDKVKEACSKHLKVAAYCTTQVERNACLFCKARKLDDKFYQKLRGQFPDAVFWQELGEILRQLQKQAAEIYNQSLIELYYEIFIKGRGFANASSVEHYLSDVCYTRAAELFKNAAIASGLRGKVKGNFRLKELKNMKSGLPTTKSDNFPIPLVRQKGGQYTGFEISSHNDDFIIKIPFGRWQVKKEIDKYRPWEKFDFEQVRKSPKPISLLLSTQRRKRNKGWSKDEGTEAEIRKVMNGDYQTSYIEVKRGSRTGEKSAWMLNLSIDVPKIDKGVDPSIIGGIDVGVKSPLVCAINNAFSRYSISDNDLFRFNKKMFARRRILLKKNRHKRAGHGAKNKLKPISILTGKSERFRKKLIERWACEIADFFTKNKVGTVQMENLESMKRKEDSYFNIRLRGFWPYAEMQNKIEFKLKQYGIEIRKVAPNNTSKTCSKCGHLNNYFNFEYRKKNKFPHFRCEKCNFKENADYNAALNISNPKLKSTKEEP

SEQ ID NO: 2616 - protein, 726 aa, synthetic construct
SEVEFSHEYWMRHALTLAKRARDEREVPVGAVLVLNNRVIGEGWNRAIGLHDPTAHAEIMALRQGGLVMQNYRLTDATLYVTFEPCVMCAGAMIHSRIGRVVFGVRNSKRGAAGSLMNVLNYPGMNHCVEITEGILADECAALLCDFYRMPRRVFNAQKKAQSSFNSGGSSGCGSGSETPGTSESAAPKSSGGGSSGSAKNTITKTLQLRIVRPYNSAEVEKIVADEKNNREKIALEKNKDKVKEACSKHLKVASYCTTQVERNACPFCKARKLDDKFYQKLRGQFPDAVFWQELGEILRQLQRQAAEIYNQSLIELYYEIFIKGRGFANASSVEHYLSDVCYTRAAELFRNAAIASGLRGKVKSNFRLKELKNMKSGLPTTKSDNFPIPLVKQKGGQYTGFEISSHNDDFIIKIPFGRWQVKKEINKHRPWEKFDFEQVRKSPKPISLLLSTQRRKRNKGWSKDEGTEAEIRKVMNGDYQTSYIEVKRGSKIGEKSAWMLNLSIDVPKIDKGVDPSIIGGIDVGVKSPLVCAIDNALSRYSISDNDLFHFNKKMFARRRILLKKNRHRRAGHGAKNKLKPISILTEKSKRFRKKLIERWACEIADFFIKNKVGTVQMENLESMKRKEDSYFNIRLRGFWPYAEMQNKIEFKLKQYGIEIRKVAPNNTSKTCSKCGHLNNYFNFEYRKKNKFPHFKCEKCNFKENADYNAALNISNPMLKSTKEEP

SEQ ID NO: 2617 - protein, 726 aa, synthetic construct
SEVEFSHEYWMRHALTLAKRARDEREVPVGAVLVLNNRVIGVGWNRAVGLHDPTAHAEIMALRQGGLVMQNYRLIDATLYVTFEPCVMCAGAMVHSRIGRVVFGVRNSKRGAAGSLMNVLDYPGMGHRVEITEGILADECAALLCDFYCMPRQVFNAQKRAQSSINSGGSSSGSSGSDTPGTSESATPESSGGGSSGSAKNTITKTLQLRIVRPYNSAEVEKIVADEKNNREKIALEKNKDKVKEACSKHLKVASYCTTQVERNACLFCKARKLDDKFYQKLRGQFPDAVFWQEIGEIFRQLQKQAAEIYNQSLIELYYEILIKGKGFANASSVEHYLSDVCYTRAAELFKNAAIASGLRGKVKSNFRLKELKNMKSGLPTTKSDNFPIPLVKQKGGQYTGFEISNHNSDFIIKIPFGRWQVKKEIDRYRPWEKFDFEQVRKSPKPISLLLSTQRRKRNKGWSKDEGTEAEIKRVMNGDYQISYIEVKRGSRIGEKSAWMLSLSVDVPKIDKGVDPSIIGGIDVGVKSPLVCAINNALSRYSISDNDLFHFNKKMFARRRILLRNNRHKRAGHGAKSKLKPITILTEKGERFRKKLIERWACEIANFFVKNKVGTVQMENLESMKRKEDSYFNVRLRGFWPYAEMQNKIEFKLKQYGIEIRKVAPNNTSKTCSKCGHLNNYFNFEYRKKNKFPHFKCEKCSFKENADYNAALNISNPKLKSTKEEP

SEQ ID NO: 2618 - protein, 725 aa, synthetic construct
SEVEFSHEYWMRHALTLAKRARDEREVPVGAVLVLNNRVIGEGWNRTTGLHDPTAHAEIMALRQGGLVMQNHRLVDATLYVTFEPCVMCAGALVHSRIGRVVFGVRNSKRGAAGSLMNVLDYPGMGHRVEITEGILADECAALLCDFYCMPRQVFNAQKRAQSSINSGGSSGGSSGSETPGTSESATPESSGGGSSGSAKNTITKTLQLRIVRPYNSAEVEKIVADEKNNREIALEKNKDKVKEACSKHLKVASYCTTQVERNACPFCKARKLDDKFYQKLRGQFPDAVFWQEIGEIFRQLQKQAAEVYNQSLVELYYEILIKGKGFANASSVEHYLSDVCYTRAAELFKNAAIASGLRGKVKSNFRLKELKNMKSGLPTTKSDNFPIPLVKQKGGQYTGFEISSHNSDFIIKIPFGRWQVKEEIDKYRPWEKFDFEQVRKSPKPISLLLSTQRRKKNKGWSKDEGTEAEIRRVMNGDYQTSYIEVKRGSKIGEKSAWMLNLSIDVPKIDKGVNPSIIGGIDVGVKSPLVCAINNSSSRYSICDNDLFRFNKKMFARRRILLKKNRHRRAGHGAKNKLKPITILTEKSKRFRKKLIERWACEIADFFIKNKVGTVQMENLESMKRKEDSYFNIRLRGFWPYAEMQNKIEFKLKQYGIKIRKVAPNNTSRTCSKCGHLNNYFSYEYRKKNKFPHFKCEKCNFKEDADYNAALNISNPKLKGTKEEL

SEQ ID NO: 2619 - protein, 726 aa, synthetic construct; identical to SEQ ID NO: 684

SEQ ID NO: 2620 - protein, 726 aa, synthetic construct
SEDEFSHEYWMRHALTLAKRARDEREVPVGAILVLNNRVIGEGWNRAIGLHDPTAHAEIMALRQGGLVMQNYRLIDATLYVTFEPCVMCAGAMIHSRIGRVVFGVRNNKHGAAGSLVNVLNYPGMNHRVEITEGILADECAALLCDFYRMPRQVFNARKKAQSSINSVGSSGGGSGSETPSTGESATPESSGGSSGGPAKNTITKTLKLRVVRPYNSAEVEKIVADEKNNREKIALEKNKDKVKEACSKHLKVAAYCTTQVERNACLFCKARKLDDKFYQKLRGQFPDAVFWQEVGEIFRQLQKQAAEIYNQSLIELYYEIFIKGKGFANASSVEHYLSDVCYTRAAELFKNAAIASGLRGKVKSNFRLKELKNMKSGLPTTKSDNFPIPLVKQKGGQYTGFEISNHNSDFIIKIPFGRWQVKKEIDKYRPWEKFDFAQVRKSPKPISLLLSTQRRKRNRGWSKDEGTEAEIRKVMNGDYQTSYIEVKRGSKIGEKSAWMLNLSIDVPKIDKGVDPSIIGGIDVGVKSPLVCAINDAFSRYSISDNDLFHFNKKMFARRRILLKKSKHKRAGHGAKNKLKPITILTKKSGRFRKKLIERWACEIADFFIKNKVGTVQMENLESMKRKEDSYFNIRLRGFWPYAEMQNKIEFKLKQYGIKIRKVAPNNTSKTCSKCGHLNNYFNFEYRKKNKFPHFKCEKCNFKENADYNAALNISNPKLKSTKEEP

SEQ ID NO: 2621 - protein, 726 aa, synthetic construct
SEVEFSHEYWMRHALTLAKRARDECEVPVGAILVLNNRVIGEGWNRAIGLHDPTAHAEIMALRQGGLVMQNYRLIDATLYVTFEPCVMCAGAMIHSRIGRVVFGVRNSKHGAAGSLVNVLNYPGMNHRVEITEGILADECAALLCDFYRMPHQVLNAQKKAQSSINSGGSSGGSSGSETPGTSGSATPEGSGGSSGGSAKSTITKTLKLRIVRPYNSAEVEKIVADEKNNREKIALEKNKGKVKEACSKHLKVAAYCTTQVERNACLFCKARRLDDKFYQKLRGQFPDAVFWQETGEIFRQLQRQAAEIYNQSLIELYYEIFIKGRGFANASSVEHYLSDVCYTRAAELFKNAAIASGLRGKVKSNFRLKELKNMKSGLPTTKSDNFPIPLVKQKGGQYTGFEISSHNDDFIIKIPFGRWQVKKEIDKYRPWEKFDFEQVRKSPKPISLLLSTQRRKRNKGWSKDEGTEAEIKRVMNGDYQTSYIEVKRGSKVGEKSAWMLNLSIDVPKIDKGVDPSIIGGIDVGVKSPLVCAINNAFSRHSISDNDLFHFNKKMFARRRILLKKNKHKRAGHGAKNKLKPITILTGKSVRFRKKLIERWACEIADFFIKNKVGTVQMENLESMKRKEDSYFNIRLRGFWPYAEMQNKIEFKLKQYGIGVRKVTPNNTSKTCSRCGHLNNYFSFEYRKKNKFPHFKCEKCNFKEDADYNAALNISNPKLKSTREEP

SEQ ID NO: 2622 - protein, 726 aa, synthetic construct
SEVEFSHEYWMRHALTLAKRARDEREVPVGAVLVLNNRVIGEGWNRAIGLHDPTAHAEIMALRQGGLVMQNYRLSDATLYVTFEPCVMCAGAMIHSRIGRVVFGVHNSKRGAAGSLMNVLNYPGMNHCVEITEGILVDECAALLCDFYRMPRQVLSAQKKAQSSVSSGGSSGGSCGSETPGASGSVTPKSSVGSSAGSTKNTITKTLKLRIVRPYNSAEVEKIVVDEKNNREKVALERNKDKVKEACSEHLKVAAYCTTQVERSACLFCKARKLDDKFYQKLRGQFPDAVFWQEIGEIFRQLQKQAAEIYNQSLIELYYEIFIKGKGFANASSVEHYLSDVCYTRAAELFKNAAIASGLRGKVKSNFRLKELKNMKSGLPTTKSDNFPIPLVRQKGGQYTGFEISNHDGDFIIKIPFGRWQVKKEINKHRPWEKFDFEQVRKSPKPISLLLSTQRRKRNKGWSKDEGTEAEIRKVMNGDYQTSYIEVKRGSKIGEKSAWMLNLSIDVPKIDKGVDPGIIGGIDVGVKSPLVCAINSALSRYSISDNDLFHFNKKMFARRRILLRKNRHKRAGHGAKNKLKPITMMTEKSKRFRKKLIERWACEIADFFIKNKVGTVQMENLESMKRKEDSYFNIRLRGFWPYAEMQNKIEFKLKQYGIVVRKVAPNNTSKTCSKCGHLNNYFNFEYRKKNKFPHFKCEKCNFKEDADYNAALNISDPKLKSSKGEP

SEQ ID NO: 2623 - protein, 726 aa, synthetic construct
SEVEFSHEYWMRHALTLAKRARDEREVPVGAVLVLNNRVIGEGWNRAIGLHDPTAHAEIMALRQGGLVMQNYRLVNATLYVTFEPCVMCAGAMIHSRIGRVVFGVRNSKRGAAGSLMNVLNYPGMNHCVEITEGILVDECAALLCDFYRMPRQVLNAQKRAQSSINSGGSSGCSSGSETPGTSESATPESSGGGSSGSAKNTITKTLQLRIVRPYNSAEVEKIVADEKNNREKIALEKNKDKVKEACSKHLKVASYCTTQVERSACPFCKARKLDDKFYQKLGGQFPDAVFWQELGEILRQLQKQAAEIYNQSLIELYYEIFIKGRGFANASSVEHYLSGVCYTRAAELFKNAAIASGLRGKVKSNFRLKELKNMKSGLPTTKSDNFPIPLVRQKGGQYTGFEISSHNDDFIIKIPFGRWQVKKEIDKYRPWEKFDFEQVRKSPKPISLLLSTQRRKRNKGWSKDEGTEAEIRKVMNGDYQTSYIEVKRGSKIGEKSAWMLNLSIDVPKIDKGVDPSIIGGIDVGVKSPLVCAISNAFSRYSISDNDLFRFNKKMFARRRILLKKNRHKRAGHGAKNKLKPISILTEKSERFRKKLIERWACEIADFFIKNKVGTVQMENLESMKRREDSYFNIRLRGFWPYAKMQNKIEFKLKQYGIEIRKVAPNNTSKTCSKCGHLNNYFNFEYRKKNKFPHFKCEKCNFKESADYNAALNISNPKLKSTKEEP

SEQ ID NO: 2624 - protein, 726 aa, synthetic construct
SEGEFSHEYWMRHALTLAKRARDGREVPVGAVLVLNNRVIGEGWNRAIGLHDPTAHAEIMALRQGGLVMQNYRLIDATLYVTFEPCVMCAGAMVHSRIGRVVFGVRNSKRGAAGSLMNVLDYPGMGHRVEITEGILADECAALLCDFYCMPRQVFNAQKRAQSSINSGGSSDGSSGSETPGTSESATPESSGGGSSGSAKNTITKTLQLRIVRPYNSAEVEKIVADEKNNREKIALEKNKGKVREACNKHLKVASYCTTQVERNACPFCKARKLDDKFYQKLRGQFPDAVFWQEIGEIFRQLQKQAAEIYNQSLIELYYEIFIKGKGFANASSVEHYLSDVCYTRAAELFKNAAIASGLRGKVKSNFRLKELKNMKSGLPTTKSDNFPIPLVKQKGGQYAGFEISSHNDDFIIKIPFGRWQVKKEIDKYRPWEKFDFEQVRKSPKPISLLLSTQRRKRNKGWSKDEGTEAEIRKVMNGVYQTSYIEVKRGSKIGEKSTWMLNLSIDVPKIDKGVDPSIIGGIDVGVKSPLVCAINNAFSRYSISDNDLFHFNKKMFARRRILLKKNRHKKAGHGAKNKLKPISILTEKSERFRKKLIERWACEIADFFIKNKVGTVQMENLESMKRKEDSYFNIRLRGFWPYAEMQNKIEFKLKQYGIEIRKVAPNNTSKTCSKCGHLNNYFNFEYRKKNKFPHFKCEKCDFKENADYNAALNISNPKLKSTKEEP

SEQ ID NO: 2625 - protein, 726 aa, synthetic construct
SEVEFSHEYWMRHALTLAKRARDEREVPVGAILVLNNRVIGEGWNRAIGLHDPTAHAEIMALRQGGLVMQNYRLIDATLYVTFEPCVMCAGAMIHSRIGRVVFGVRNSKHGAAGSLMNVLNYPGMNHRVEITEGILADECAALLCDFYRMPRQVFNARKKAQSSINPGGPSGSSSCSETPGASESVTPKSSGGSSTGSTKNTITKTLKLRIVRPYNSAEVEKIVADEKNSREKIALEKNRDKVKEACSEHLKVAAYCTTQVERNACLFCKARKLDDRFYQKLRGQFPDAVFWQEIGEIFRQLQKQAAEIYNQSLIELYYEIFIKGKGFANASSVEHYLSDVCYTRAAELFKNAAIASGLRGKVKSNFRLKELKNMKSGLPTTKSDNFPIPLVRQKGGQYTGFEISNHDGDFIIKIPFGRWQVKKEICKHRPWEKFDFEQVRKSPKPISLLLSTQRRKRNKGWGKDEGTEAEIRKVMNGDYRTSYIEVKRGSKIGEKSAWMLNLSIDVPKIDKGVDPSIIGGFDVGVKSPLVCAINNALSRYSISDNDLFHFNKKMFARRRILLRKNRHKRAGHGARNKLKPITVLTEKSERFRKKLIERWACEIANFFIKNKVGTVQMENLESMKRREDSYFNIRLRGFWPYAEMQSKIEFKLKQYGIKIRKVAPNNTSKTCSKCGHLNNYFNFEYRKKNKFPHFKCEKCNFKENADYNAALNISNPKLKSTKEEP

SEQ ID NO: 2626 - protein, 726 aa, synthetic construct
SEVEFSHEYWMRRALTLAKRARDEREVPVGAVLVLNNRVIGVGWNRAVGLHDPTAHAEIMALRQGGLVMQNYRLVEATLYVTFEPCIMCAGAMIHSRIGRVVFGVRNSKRGAAGSLTNVLNHPGMNHRVEITEGILADECAALLCDYYRMPRQVFNARKKAQPSINSGGSSDGGSGSETPGTSESATPESSGGSSGGSAKNTITKALKLRIVRPYNSAEVEKIVADEKNNRERIALEKNKDKVKEACSKHLKVAAYCTTQVERNACLFCKARKLDDKFYQKLRGQFPDAVFWQEIGEIFRQLQKQAAEIYNQSLIELYYEIFIKGKGFANASSVEHYLSDVCYTRAAELFKNAAIASGLRGKVKSNFRLKELKNMRSGLPTTKSDNFPIPLVKQKGGQYAGFEISSHNDDFIIKIPFGRWQVKKEIDKYRPWEKFDFEQVRKSPKPISLLLSTRRRKRNKGWSKDEGTEAEIRKVMNGDYQTSYIEVKRGSKIGEKSAWMLNLSIDVPKIDKGVDPSIIGGIDVGVKSPLVCAINNAFGRYSISDNDLFHFNKKMFARRRILLKRNRHKRAGHGAKNKLKPITILTEKSKRFRRKLIERWACEIADFFIKNKVGTVQMENLESMKRKEDSYFNIRLRGLWPYAEMQDKIEFKLKQYGIEIRRVAPNNTSKTCSRCGHLNNYFNFEYRRKNKFPHFKCEKCNFKENADYNAALNISNPKLKSTKEEP

SEQ ID NO: 2627 - protein, 726 aa, synthetic construct
SEVEFSHEYWMRHALTLAKRARDEREVPVGAILVLNNRVIGEGWNRAVGLHDPTAHAEIMALRQGGLVMQNYRLIDATLYVTFEPCVMCAGAMIHSRIGRVVFGVRNSKHGAAGSLVNVLNYPGMNHRVEITEGILADECAALLCDFYRMPRQVFSARKKAQSSINPGGSSGGSSGSKTPGTSESATPESSGGSSGGSAKNSITKTLKLRIVRPYNSAEVEKIVADEKNNREKIALEKNKGKVKEACSKHLKVATYCTTQVERNACLFCKARKLDDKFYQELRGQFPDAVFWQELGEIFRQLQKQAAEIYNQSLIELYYEIFIEGKGFANASSVEHYLSDVCYTRAAELFKNAAIASGLRGKVKGNFRLKELKSMKSGLPTTKSDNFPIPLVRQKGGQYTGFEISNHNGDFIIKIPFGRWQVKKEISKHRPWEKFDFEQVRKSPKPISLLLSTQRRKRNKGWGKDEGTEAEIRKVMNGDYQTSYIEVKRGSKIGEKSAWMLNLSIDVPKVDKGVDPNIIGGIDVGVKSPLVCAINNALSRYSISDNDLFHFNKKMFARRRILLRKNRYKRAGHGARNKLKPITVLTEKSERFRKKLIERWACEIANFFIKNKVGTVQMEDLESMKRREDSYFNIRLRGFWPYAEMQSKIEFKLKQYGIKIRKVAPNNTSKTCSKCGHLNNYFSFEFRKKNKFPHFKCEKCNFKEDADYNAALNISNPKLKSTKEEP

SEQ ID NO: 2628 - protein, 726 aa, synthetic construct
SEVEFSHEYWMRHALTLAKRARDGREVPVGAVLVLNNRVIGEGWNRAIGLHDPTAHAEIMALRQGGLVMQNYRLIDATLYVTFEPCVMCAGAMVHSRIGRVVFGVRNGKRGAAGSLMNVLDYPGMGHRVEITEGILADECAALLCDFYCMPRQVFNAQKRAQSSINSSGSSGGSSGSETPGTSESATPESSGGSSGGSAKNTITKTLKLRIVRPYNSAEVEKIVADEKNNREKIALEKNKDKVKEACSKHLKVASYCTTLVERNACLFCKARELDDKFYQKLRGQFPDAVFWQEVGEIFRQLQKQAAEIYNQSLIELYYEIFIKGKGFANASSVEHYLSDVCYTRAAELFKNAAIASGLRGKVKSNFRLKELKNMKSGLPTTKSDNFPIPLVKQKGGQYTGFEISNRNSDFIIKIPFGRWQVKREIDKYRPWEKFDFEQVRKSPKPISLLLSTQRRKRNKGWSKDEGTEAEIRKVMNGDYQTSYIEVKRGSKIGEKSAWMLNLSIDVPKIDKGVDPSIIGGIDVGVKSPLVCAINNAFSRYSISDNDLFRFNKKMFARRRILLKKNRHKRAGHGAKNKLRPISILTGKGERFRKKLIERWACEIADFFIRNRVGTVQMENLESMKRKEDSYFNIRLRGFWPYAEMQNKIEFKLEQYGIVVRKVAPNNTSKTCSKCGHLNNYFNFEYRKKNKFPHFKCEKCNFKENADYNAALNISNPKLKSTKGEP

SEQ ID NO: 2629 - protein, 726 aa, synthetic construct
SEVEFSHEYWMRHALTLAKRARDEREVPVGAILVLNNRVIGEGWNRAIGLHDPTAHAEIMALRQGGLVMQNYRLIDATLYVTFEPCVMCAGAMIHSRIGRVVFGVRNSKHGAAGSLVNVLNYPGMNHRVEITEGILADECAALLCDFYRMPRQVFNARKKAQSSINPSGSSGGSSGSVTPGTSESATPESSSGGFGGSAKNTITKTLQLRIVRPYNSAEVEKIVADEKNNREKIALEKNKDKVKEACSKHLKVASYCTTQVERNACLFCKARKLDDKFYQKLRGQFPDAVFWQELGGIFRQLQKQAAEIYNQSLIELYYEIFIKGKGFANASSVEHYLSDVCYTRAAELFKNAAIASGLRGKVKSNFRLKELKNMKSGLPTTKSDNFPIPLVKQKGGQYTGFEISSHNDDFIIKIPFGGWQVRKVIDKYRPWEKFDFEQVRKSPKPISLLLSTQRRKRNKGWSKDEGTEAEIRKVMNGDYQTSYIEVRRGSKTGEKGAWMLNLSIDVPKIDKGVDPSVIGGIDVGVKSPLVCAINNAFSRFSISDNDLFHFNKKMFARRRILLKKNGRKRAGHGAKNKLKPITILTEKSKRFRKKLIERWACEIAGFFIKNKVGTVQMENLESMKRKEDSYFNIRLRGFWPYAEMQNKIEFKLKQYGIEIRKVAPNNTSKTCSKCGHLNDYFNFEYRKKNKFPHFKCEKCNFKENADYNAALNISSPKLKSTREEP

SEQ ID NO: 2630 - protein, 726 aa, synthetic construct
SEVEFSHEYWMRHALTLAKRARDEREVPVGAVLVLNNRVIGEGWNRAIGLHDPTAHAEIMALRQGGLVMQNYRLTDATLYVTFEPCVMCAGAMIHSRIGRVVFGVRNSKHGAAGSLVNVLNYPGMNHRVEITEGILADECAALLCDFYRMPRQVLNAQKKAQSSISSGGSSGGSSGGETPGASESVTPKDSGGSSADSTKNTITKTLKLRIVRPYNSAEVEKIVADEKNSREKIALEKNKDKVKEACREHLKVASYCTTQVERSACPFCKARKLDDKFYQKLGGQFPDAVFWQELGGIFRQLQKQAAEIYNQSLIELYYEIFIKGRGFANASSVEHYLSDVCYTRAAELFKNAAIASGLRGKVKSNFRLKELKNMKSGLPTTKSDNFPIPLVKQKGGQYTGFEISSHNGDFIIKIPFGRWQVKEEIDKFRPWEKFDFEQVRKSPKPISLLLSTQRRKKNKGWSKDEGTEAEIRRVMNGDYQTSYIEVRRGSKIGEKSAWMLNLSIDVPKIDKGVDPSIIGGIDVGVKSPLVCAINNAFSRYSISDNELFHFNKKMFARRRILLKKNRHKRAGHGAKNKLKPITVLTEKSERFRKKLIERWACEIANFFIKNKVGTVQMENLESMKRREDSYFNIRLRGFWPYAEMQNKIEFKLKQYGIEVRKVAPNNTSKTCSKCGHLNNYFNFEFRKKNKFPHFKCGKCNFKENADYNAALNISNPKLKSTKEEP

SEQ ID NO: 2631 - protein, 726 aa, synthetic construct
SEVEFSHEYWMRHALMLAKRARDEREVPVGAVLVLNNRVIGEGWNRAIGLHDPTAHAEIMALRQGGLAMQNYRLVDATLYVTFEPCVLCAGAMVHSRIGRVVFGVRNSKRGAAGSLMNVLNHPGMNHRVEITGGILADECAALLCDFYRMPRQVFNAQKKARSNINSGGSSGGSSGSETLGTSESATPESSGGSSGGSAKNTITKTLQLRIVRPYNSAEVEKIVADEKDNRERVALEKNKDKVKEACSEHLKVAAYCTTQVERNACLFCKARKLDDKFYQKLRGQFPDAVFWQEISEIFRQLQKQAAEIYNQSLVELYYEIFVKGKGFANASSVEHYLSDVCYTRAAELFKNAAIASGLRGKVKGNFRLKELKNMKSGLPTTKSDNFPIPLVKQKGGQYTGFEISSHNSDFIIKIPFGRWQEKEEIDKYRPWEKFDFEQVRKSPKPISLLLSTQRRKKNKGWSKDEGTEAEIRRVMNGDYQTSYIEVKRGSKIGEKSAWMLNLSIDVPKIDKGVDPSIIGGIDVGVKSPLVCAINNAFSRYSISDNDLFHFNKKMFARRRILLKKNRHRRAGHGAKNKLKPITILTEKSVRFRKKLIERWACEIANFFIKSKVGTVQMENLESMKRKEDSYFNIRLRGFWPYAEMQNKIEFKLKQYGIEIRKVAPDNTSKTCSKCGHLNNYFNFEYRKRNKFPHFKCEKCNFKEDADYNAALNISNPKLKGTKEEL

SEQ ID NO: 2632 - protein, 726 aa, synthetic construct
SEDEFSHEYWMRHALTLAKRARDEREVPVGAVLVLNNRVIGEGWNRAIGLHDPTAHAEIMALRQGGLVMQNYRLVDATLYVTFEPCVLCAGAMVHSRIGRVVFGVRNSKRGAAGSLMNVLNYPGMNHRVEITEGILADECAALLCDFYRMPRRVFNARKKARSNINPSGSSGGSSGSETPGTSESATPESSGGSSGGSAKNTITKTLKLRIVRPYNSAEVEKIVADEKNNREKIALEKNKDKVKEACSEHLKVAAYCTTQVERNACLFCRARKLDDKFYQKLRGQFPDAVFWQEIGEIFRQLQKQAAEIYNQSLIELYYEIFIKGKGFANASSVEHYLSDVCYTRAAELFKNAAIASGLRGKVKSNLRLKELKNMKSGLPTTKSDNFPIPLVKQKGGQYTGFEISSHNDDFIIKIPFGRWQAKKEIDKYRPWEKFDFEQVRKSPKPISLLLSTQRRKRNRGWSKDEGTEAEIRKVMNGDYQTSYIEVKRGSKIGEKSAWMLNLSIDVPKIDKGVDPSIIGGIDVGVKSPLVCAINNAFSRYSISDNDLFRFNKKMFARRRILLGKNRHKRAGHGVKNKLKPITILTEKSGRFRKKLIERWACEIADFFVKNKVGTVQMENLESMKRKEDSYFNIRLRGFWPYAEMQNKIEFKLRQYGIKVRKVAPNNTSKTCSKCGHLNNYFSFEYRKKNKFPHFKCEKCNFKENADYNAALNISNPKLKGTKEEP

SEQ ID NO: 2633 - protein, 726 aa, synthetic construct
SEVEFSHEYWMRHALTLAKRARDEREVPVGAVLVLNNRVIGVGWNRAIGLHDPTAHAEIMALRQGGLVMQNYRLTDATLYVTFEPCVMCAGAMVHSRIGRVVFGVRNSKRGAAGSLMNVLNYPGMSHCVEITEGILVDECAALLCDFYRMPRQVLNAQKKAQSSISSGGSSGGSGGGETPGASESVTPKSFGGSPGGPAKNTITKTLKLRIVRPYNSTEVEKIVADEKNNREKIALEKNKDKVKEACSKHLKVAAYCTTQVERNACLFCKARKLDDKFYQKLRGQFPDAVFWQEIGEIFRQLQKQAAEIYNQSLIELYYEIFIKGKGFANASSVEHYLSDVCYSRAAELFKNAAVASGLRGKVKSNFRLKELKNMKSGLPTTKSDNFPIPLVKQKGGQYTGFEISSHNDDFIIKIPFGRWQVKEEIDKYRPWEKFDFEQVRKNPKPISLLLSTQRRKRNKGWSKDEGTEAEIRKVMNGDYQTSYIEVKRGSKTGEKSAWMLNLSIDVPKIDKGVDPGIIGGIDVGVKSPLVCAINNASSRYSIGDNDLFHFNKKMFARRRILLKKNRHKRAGHGAKNKLKPLTILTEKSRRFRKKLIERWACEIADFFIKNKVGTVQMESLESMRRKEDSYFNIRLRGFWPYAEMQNKIEFKLKQYGIEIRKVAPNNTSKTCSKCGHLNNYFNFEYRKKNKFPHFKCEKCNFKENADYNAALNISNPELKGTKEEP

SEQ ID NO: 2634 - protein, 726 aa, synthetic construct
SEVEFSHEYWMRHALTLAKRARDEREVPVGAILVLNNRVIGEGWNRAIGLHDPTAHAEIMALRQGGLVMQNYRLIDATLYVTFEPCVMCAGAMIHSRIGRVVFGVRNNKHGAAGSLVNVLNYPGMNHRVEITEGILADECAALLCDFYRMPRQVFNARKKAQSSINPGGSSGGSSGSETPGTSESATPESSGGSSGSSAKNTITKTLKLRIVRPYNSAEVEKIVADEKNNREKIALEKNKDKVKEACSKHLKVAAYCTTQVGRNACLFCKARRLDDKFYQKLRGQFPDAVFWQEIGEIFRQLQKQAAEVYNQSLVELYYEILIKGKGIANASSVEHYLSDVCYTRAAELFKNAAIASGLRNKIKSNFRLKELRNMKSGLPTTKSDNFPIPLVRQKGGQYTGFEISNHDGDFIIKIPFGRWQVKKEINKHRPWEKFDFEQVRRSPKPISLLLSTQRRKRNKGWSKDEGTEAEIRKVMNGDYQTSYIEVKRGSKIGEKSAWMLNLSIDVPKIDKGVNPSIIGGIDVGVKSPLVCAINDSSSRYSICDNDLFRFNKKMFARRRILLKKNRHKRAGHGAKNKLKPISILTERSKRFRKKLIERWACEIADFFIKNKVGTVQMENLESMKRKEDSYFNIRLRGFWPYAEMQNKIEFKLKQYGIEIRKVAPNNTSKTCSKCGHLNNYFNFEYRKMNKFPHFKCERCNFKENADYNAALNISNPKLKSTKEEP

SEQ ID NO: 2635 - protein, 726 aa, synthetic construct
SEVEFSHEYWMRHALTLAKRARDEREVPVGAVLVLNNRVIGEGWNRAIGLHDPTAHAEIMALRQGGLVMQNYRLTDATLYVTFEPCVMCAGAMIHSRIGRVVFGVRNSKRGAAGSLMNVLNYPGMNHRVEITEGILVDECAALLCDFYRMPRQVFNAQKKAQSTINPGGSSGGSSGSETPGTSESATPESSGGSSGGSAKNTVTKTLKLRIVRPYNSAEVEKIVADEKNNREKIALEKNKDKVKEACSKHLKVAAYCTTQVERNACLFCKARKLDDKFYQKLRGQFPDAVFWQEIGEIFRQLQKQAAEIYNQSLIELYYEIFIKGKGFANASSVEHYLSGVCYTRAAELFKNAAIASGLRGKVKSNFRLKELKNMKSGLPTTKSDNFPIPLVKQKGGQYTGFEISSHNDDFIIKIPFGRWQVKKEINKYRPWEKFDFEQVRKSPKPISLLLSTQRRKRNKGWSKDEGTEAEIRKVMNGGYQTSYIEVKRGGKIGEKSAWMLSLSIDVPKVDKGVDPSIIGGIDVGVKSPLVCAINNAFSRYSISDNDLFHFNKKMFARRRILLKKTRHKRAGHGAKNKLKPISILTEKSERFRKKLIERWACEIADFFIKNKVGTVQMENLESMKRREDSYFNIRLRGFWPYAKMQNKIEFKLKQYGIEIRKVAPNNTSKTCSKCGHLNNYFNFEYRKKNKFPHFKCEKCNFKESADYNAALNISNPKLKSTKEEP

SEQ ID NO: 2636 - protein, 725 aa, synthetic construct
SEVEFSHEYWMRRALTLAKRARDEREVPVGAVLVLNNRVIGVGWNRAVGLHDPTAHAEIMALRQGGLVMQNYRLIDATLYVTFEPCVMCAGAMIHSRVGRVVFGVRNSKHGAAGSLMNVLNYPGMNHRVEITEGILADECAALLCDFYRMPHRVFNGRKKAQSSINPGGSSGGSSGSETPGTRESATPSSGGSSGGSAKNTITKTLQLRIVRPYNSAEVEKIVADEKSNREKVALEKNKDKVKEACSKHLKVASYCTTQVERNACLFCKARKLDDKFYQKLRGQFPDAVFWQELGEILRQLQKQAAEIYNQSLIELYYEIFIKGRGFANASSVEHYLSDVCYTRAAELFKNAAIASGLRGKVKSNFRLKELKNMKSGLPTTKSDNFPIPLVKQKGGQYTGFEISSHNDDFIIKIPFGRWQVKKEIDKYRPWEKFDFEQVRKSPKPISLLLSTQRRKRNKGWSKDEGTEAEIRKVMNGEYQTSYIEVKRGSKTGEKSAWVLNLSIDVPKIDKGVDPSIIGGIDVGVKSPLVCAINNALSRYSISDNDLFRFNKKMFARRRILLKKNRHKRAGHGAKNKLKPISILTGKSERFRKKLIERWACEIADFFIKNKVGTVQMENLESMKRKEDSYFNIRLRGFWPYAEMQNKIEFKLKQYGIEIRKVAPNNTSKTCSKCGHLNNYFNFEYRKKNKFPHFKCEKCNFKENADYNAALNISNPRLKSTNEEP

SEQ ID NO: 2637 - protein, 726 aa, synthetic construct
SEVEFSHEYWMRHALTLAKRARDEREVPVGAVLVLNNRVIGEGWNRAIGLHDPTAHAEIMALRQGGLVMQNYRLTDATLYVTFEPCVMCAGAMIHSRIGRVVFGVRNSKRGAAGSLMNVLNYPGMNHCVEITEGILVDECAALLCDFYRMPPQVLNARKKAQSSISSGGSSGGSNGSETPGTSESATPECSGGGSSGSAKNTITKTLQLRIVRPYNSAEVEKIVADEKNNREKIALEKNKDKVKEACSKHLKVASYCTTQVERNACPFCKARKLDDKFYQKLRGQFPDAVFWQELGEILRQLQKQAAEIYNQSLIELYYEIFIKGRGFANASSVEHYLSDVCYTRAAELFKNAAIASGLRGKVKSNFRLKELKNMKSGLPTTKSDNFPIPLVKQKGGQYTGFEISNHNDDFIIKIPFGRWQAKKEIDKYRPWEKFDFEQVRKSPKPISLLLSTQRRKRNKGWSKDEGTEAEIRKVMNGDYQTSYIEVKRGSKTGEKSAWMLNLSIDVPKIDKGVDPCIMGGIDVGVKSPLVCAIHNAFGRYSISDNDLFHFNKKMFARRRILLKENGHKRAGHGAKNKLKPLTIMTEKSKRFRKKLIERWACEIADFFIKNKVGTVQMENLESMKRKEDSYFNIRLRGFWPYAEMQNKIEFKLKQYGIVVRKVAPNNTSKTCSMCGHLNNYFSFEYRKRNKFPHFKCEKCNFKENADYNAALNISNPKLKGTKEEP

SEQ ID NO: 2638 - protein, 726 aa, synthetic construct
SEVEFSHEYWMRHALTLAKRARDEREVPVGAVLVLNNRVIGEGWNRTTGLHDPTAHAEIMALRQGGLVMQNYRLTDATLYVTFEPCVMCAGAMVHSRIGRVVFGARNSKRGAAGSLMNILNYPGMNHRVEITEGILADECAALLCDFYRMPRQVFSARKKAQSSINSGGSSGGSGGGETPGASESVTPKNSGGSSSGSAKNTITKTLQLRIVRPYNSAEVEKIVADEKSNREKIALEKNKDKVREACSKHLKVASYCTTQVDRNACPFCKARKLDDKFYQKLRGQFPDAVFWQELGEILRQLQKQAAEIYNQSLIELYYEIFIKGKGIASASRVGHYLSDVCYTRAAELFKNAAIASGLRGKIKSNFRLKELRNMKSGLPTTKSDNFPIPLVKQKGGQYTGFEINSHNDDFIIKIPFGRWQVKKEIDKYRPWEKFDFEQVRKSPKPISLLLSTQRRKRNKGWSKDEGTEAEIRKVMNGDYQTSYIEVKRGSKIGEKSAWMLNLSIDVPKIDKGVDPSIIGGIDVGVKSPLVCAINNAFSRYSISDNDLFHFNKKVFARRRILLKKNRHKRAGHGAKNKLKPISILTGKSERFRKKLIERWACEIADFFIKNKVGTVQMENLESMKRKEDSYFNIRLRGFWPYAEMQNKIEFKLKQYGIEIRKVAPNNTSKTCSKCGHLNNYFNFEYRKKNKFPHFKCEKCSFKENADYNAALNISNPKLKSTKEEP

SEQ ID NO: 2639 - protein, 725 aa, synthetic construct
SEVEFSHEYWMRHALTLAKRARDEREVPVGAVLVLNNRAIGEGWNRAIGLHDPTAHAEIMALRQGGLVMQNYRLTDATLYVTFEPCAMCAGAMIHSRIGRVVFGVRNSKRGAAGSLMNVLNYPGMNHRVEITEGILTDECAALLCDFYRMPHQVLNAQKKAQSSINSGGSSGGSSGSETPGTSGSATPEGSGGSSGGSAKNTITKTLKLRIVRPYNSAEVEKIVADEKSNREIALEKNKGKVKEACSKHLKVAAYCTTQVERNACLFCRARRLDDKFYQKLRGQFPDAVFWQEIGEIFRQLQKQAAEIYNQSLVELYYEIFIKGKGIANASSVEHYLSDVCYTRAAELFKNAAIASGLRNKIKSNFRLKELRNMKSGLPTTKSDNFPIPLVRQKGGQYTGFEISNHNSDFIIKIPFGRWQVKKEIDKYRPWEKFDFAQVRKSPKPISLLLSTQRRKRNKGWSKDEGTEAEIRRVMNGDYQTSYIEVKRGSKIGEKSAWMLNLSIDVPKIDKGVDPSIVGGIDVGVKSPLVCAINNALSRYSICDNDLFHFNKKMFARRRILLRNNRHKRAGHGAKSKLKPITILTEKGERFRKKLIERWACEIANFFVKNKVGTVQMENLESMRRKEDSYFNVRLRGFWPYAEMQNKIEFKLKQYGIEIRKVAPNNTSKTCSRCGHLNNYFNFEYRRKNKFPHFKCERCNFKENADYNAALNISNPKLKSTKEEP

SEQ ID NO: 2640 - protein, 726 aa, synthetic construct
SEVEFSHEYWMRHALTLAKRARDEREVPVGAVLVLNNRVIGEGWNRAIGLHDPTAHAEIMALRQGGLVMQNYRLIDATLYVTFEPCVLCAGAMVHSRIGRVVFGVRNSKRGAAGSLMNVLDYPGMDHRVEVTEGILADECAALLCDFYRMPRQVFNARKKAQSSISPGSSSGGSSGSETPGTSESATPGSSGGGSNGSAKNTITKTLQLRIVRPYNSAEVEKIVADEKNNRERIALEKNKDKVREACNKHLKVASYCTTQVERSACPFCKARKLDDKFYQKLRGQFPDAVFWQEIGEIFRQLQKQAAETYNQSLIELYYEIFIKGKGFANASSVEHYLSDVCYTRAAELFKNAAIASGLRGKVKSNFRLKELKNMKSGLPTTKSDNFPIPLVKQKGGQYAGFEISSHNDDFIIKIPFGRWQVKKEIDKYRPWEKFDFEQVRKSPKPISLLLSTQRRKRNKGWSKDEGTEAEIRKVMNGDYQTSYIEVKRGSKTGEKSAWMLNLSIDVPKIDKGVDPSIIGGIDVGVKSPLVCAINNAFSRYSISDNDLFRFNKKMFARRRILLKKNRHKRAGHGAKNKLRPISILTGKSERFRKKLIERWACEIADFFIKNKVGTVQMENLESMKRKEDSYFNIRLRGFWPYAEMQNKIEFKLKQYGIEIRKVAPNNTSKTCSKCGHLNNYFNFEYRKKNKFPHFKCEKCNFKEDADYNAALNISNPKLKSTKEEP

SEQ ID NO: 2641 - protein, 726 aa, synthetic construct
SEVEFSHEYWMRHALTLAKRARDGREVPVGAVLVLNNRVIGEGWNRAIGLHDPTAHAEIMALRQGGLVMQNYRLIDATLYVTFEPCVMCAGAMVHSRIGRVVFGVRNSRRGAAGSLMNVLDYPGMGHRVEITEGILADECAALLCDFYCMPRQVFNAQKRAQSSINSGGSSDGSSGSETPGTSESATPESSGGGSSGSAKNTITKTLQLRIVRPYNSAEVEKIVADEKNNREKIALEKNKDKVREACNKHLKVASYCTTQVERNACPFCKARKLDDKFYQKLRGQFPDAVFWQELGEIFRQLQKQTAEIYNQSLIELYYEIFIKGKGFANASSVEHYLSDVCYTRAAELFKNAAIASGLRGKVKSNLRLKELKNMRSGLPTTKSDNFPIPLVKQKGGQYTGFEISSHNDDFIIKIPFGRWQVKKEIDKYRPWEKFDFEQVRKSPKPISLLLSTQRRKRNRGWSKDEGTEAEVKKVMNGDYQISYIEVKRGSKIGEKSAWTLNLSIDVPKIDKGVDPSIIGGIDVGVKSPLVCAISNALSRYSINDNDLFHFNKKMFARRRILLKKSKHKRAGHGAKNKLKPITILTEKSRRFRKKLIERWACEIADFFIKNKVGTVQMENLEGMKRKEDSYFNIRLRGFWPYAEMQNKIEFKLKQYGIEIRKVAPNNTSKTCSKCGHLNNYFNFEYRKKNKFPHFKCEKCSFKENADYNAALNISNPKLKSTKEEP

SEQ ID NO: 2642 - protein, 726 aa, synthetic construct
SEVEFSHEYWMRHALTLAKRARDEREVPVGAVLVLNNRVIGEGWNRAIGLHDPTAHAEIMALRQGGLVMQNYRLIDATLYVTFEPCAMCAGAMVHSRIGRVVFGVRNSKRGAAGSLMNVLNYPGMDHRVEITGGILADECAALLCDFYRMPRRVFSAQKKAQSSINSGGSSGGSSGSVTPGTSESVTPKSSGGSSAGSTKDTITKTLKLRIVRPYNSAVVEKIVADEKNSREKIALEKNKDKVKEACSEHLKVAAYCTTQVERNACLFCKARKLDDRFYQKLRGQFPDAVFWQETGEIFRQLQRQAAEIYNQSLIELYYEIFIKGKGFANASSVEHYLSDVCYTRAAELFKNAAIASGLRGKVKGNFRLKELKSMKSGLPTTKSDNFPIPLVKQKGGQCTGFEISNHNSDFIIKIPFGRWQVKKEIDKYRPWEKFDFEQVRKSPKPISLLLSTQRRRRNRGWSKDEGTEAEIRKVMNGDYQTSYIEVKRGSKAGEKSAWMLNLSIDVPKIDKGVDPCIIGGIDVGVKSPLVCAINDAFSRYSISDNDLFHFNKKMFARRRILLKKNGHKRAGHGAKNKLKPITIMTEKSKRFRKKLIERWACEIADFFIKNKVGTVQMENLESMKRKEDSYFNIRLRGFWPYAEMQNKIEFKLKQYGIVVRKVAPNNTSKTCSKCGHLNNYFNFEYRKKNKFPHFKCEKCNFKEDADYNAALNISNPKLKSTKGEP

SEQ ID NO: 2643 - protein, 726 aa, synthetic construct
SEVEFSHEYWMRHALTLAKRARDEREVPVGAVLVLNNRVIGGGWNRAIGLHDPTAHAEIMALRQGGLVMQNCRLVDATLYVTFEPCVMCAGAMIHSRIGRVVFGVRNSKRGAAGSLMNVLNYPGMNHRVEITEGILAGECAALLCDFYRMPRQVFNAQKKAQSTINSGGSSGGSSSSETPGTSGSATPEGSGGSSGGSAKNTITKTLKLRIVRPYNSAEVEKIVADEKNRREKIALEKNKDKVKEACSEHLKVAAYCTTQVERNACLFCKARKLDDRFYQKLRGQFPDAVFWQETGEIFRQLQKQAAEIYNQSLIELYYEILIKGKGFANASSVEHYLSDVCYTRAAELFKNAAIASGLRGKVKSNFRLKELKNMKSGLPTTKSDNFPIPLVKQKGGQYTGFEISSHNDDFIIKIPFGRWQVKKEIDKYRPWEKFDFEQVRKSPKPISLLLSTQRRKRNRGWSKDEGTEAEIRKVMNGDYQTSYIEVKRGSKIGEKSAWMLNLSIDVPKIDKGVDPSIIGGIDVGVKSPLVCAINNAFSRYSISDNDLFHFNKKMFARRRILLKKNRRRRAGHGAKNKLKPITILTEKSARFRKKLIERWACEIADFFIKNKVGTVQMENLESMKRREDSYFNIRLRGFWPYAEMQNKIEFKLRQFGIEIRKVAPHNTSKTCSKCGHLNNYFNFEYRRKNKFPYFKCGKCNFKEDADYNAALNISNPKLKSTKEKP

SEQ ID NO: 2644 - protein, 726 aa, synthetic construct
SEVEFSHEYWMRHALSLAKRARDEREVPVGAVLVLNNRIIGEGWNRAIGLHDPTAHAEIMALRQGGLVMQNYRLTDATLYVTFEPCVMCAGAMVHSRIGRVVFGVRNSKRGAAGSLMNVLNYPGVNHCVEITEGILVDECAALLCDFYRMPRRVLNAQKKAQSSISSGGSSGGCSGSEMPGASESVTPKSSGGSSAGSTKNTITKTLKLRIVRPYNSAEVEKIVADEKNNREKIALEKNKDKVKEACSEHLKVAAYCTTQVERSACLFCKARKLDDKFYQKLRGQYPDAVFWQEIGEIFRQLQKQAAEIYNQSLIELYYEIFIKGKGFANASSVEHYLSDVCYTRAAELFKNAAIASGLRGKVKSNFRLKELKNMRSGLPTTKSDNFPIPLVKQKGGQYTGFEISSHNDDFIIKIPFGRWQVKKEIDKYRPWEKFDFEQVRKSPKPISLLLSTRRRKRNKGWSKDEGTEAVIRKVMNGDYQTSYIEVKRGSKIGEKSAWMLNLSIDVPKIDKGVDPSIIGGIDVGVKSPLVCAINNAFSRYSISDNDLFRFNKKMFARRRILLGKNRHRRAGHGAKNKLKPISILTEKSKRFRKKLIERWACEIADFFIKNKVGTVQIENLESMRRKEDSYFNIRLRGFWPYAEMQNKIEFKLKQYGIKIRKVAPNNTSKTCSKCGHLNNYFNFEYRKKNKFPHFKCEKCNFKENADYNAALNISNPKLKSTKEEP

SEQ ID NO: 2645 - protein, 726 aa, synthetic construct
SEVEFSHEYWMRHALTLAKRARDEREVPVGAVLVLNNRVIGVGWNRAIGLHDPTAHAEIMALRQGGLVMQNYRLTDATLYVTFEPCVMCAGAMIHSRIGRVVFGVRNSKRGAAGSLMNVLNYPGMNHCVEITEGILVDECAALLCDFYRMPRQVLNAQKKAQSSISSGGSSGGSSCSETPGASESVTPKSSGGGFGSSAKNTITKTLQLRIVRPYNSAEVEKIVADEKNNREKIALEKNKDKVKEACSEHLKVAAYCTTQVERNACLFCKARKLDDRFYQKLRGQFPDAVFWQELGEIFRQLQKQAAEIYNQSLIELYYEIFIKGKGFANASNVEHYLSDVCYTRAAELFKNAAIASGLRGKVKSNFRLKELKNMKSGLPTTKSDNFPIPLVKQKGGQYTGFEISSHNDDFIIKIPFGRWQVKEEIDKYRPWEKFDFEQVRKNPKPISLLLSVQRRKRNKGWSRDEGTEAEIRKVMNGDYQTSYIEVKRGSKIGEKSAWMLNLSIDVPKIDKGVDPSVIGGIDVGVKSPLICAINNAFSRYGISDNDLFRFNKKVFARRRILLKKNRHKRAGHGTKNKLKPITILTEKSGRFRKKLIERWACEIANFFIKNKVGTVQMENLESMKRKEDSYFNIRLRGFWPYAEMQNKIEFKLKQYGIKIRKVAPNNTSKTCSKCGHLNNYFNFEYRRKYKFPHFKCEKCNFKEDADYNAALNISNPKLKSTKEEP

SEQ ID NO: 2646 - protein, 726 aa, synthetic construct
SEVEFSHEYWMRHALTLAKRARDEREVPVGAVLVLNNRVIGVGWNRAIGLHDPTAHAEIMALRQGGLVMQNYRLTDATLYVTFEPCVMCAGAMIHSRIGRVVFGVRNSKHGAAGSLVNVLNHPGMNHRVEITEGILADECAALLCDFYRMPRQVFNARKKAQSSINPGGSSGGSSGSETPGTSESATPESSGGSSGGSAKNTITKTLKLRIVRPYNSAEVEKIVADEKNNREKIALEKNKDKVKEACSKHLKVAAYCTTQVERNACLFCKARRLDDKFYQKLRGQFPNAVFWQEIGEIFRQLQKQAAETYNQSLIELYYEIFIKGKGIANASNVEHYLSDVCYTRAAELFKNAAIASGLRNKIKSNFRLKELRNMKSGLPTTKSDNFPIPLVKQKGGQYTGFEISSHNDDFIIKIPFGRWQVKKEISKHRPWEKFDFEQVRKSPKPISLLLSTQRRRRNKGWSKDEGTEAEIRKVMYGDYQTSYIEVKRGSKVGEKSAWMLNLSIDVPKIDKGVDPSIIGGIDVGVKSPLVCAINNAFSRYSISDNDLFHFNKKVFARRRILLKKNRHRRAGHGAKNKLKPITILTEKSRRFRKKLIERWACEIADFFIKNKVGTVQMENLESMKRKEDSYFNIRLRGFWPYAEMQNKIEFKLKQYGIEIRKVAPNNTSRTCSKCGHLNNYFNFEYRKKNKFPHFKCEKCNFKENADYNAALNISNPKLKSTKEEP

SEQ ID NO: 2647 - protein, 726 aa, synthetic construct
SEVEFSHEYWMRRALTLAKRARDEREVPVGAVLVLNNRVIGEGWNRAIGLHDPTAHAEIMALRQGGLVMQNYRLIDATLYVTFEPCVMCAGAMVHSRLGRVVFGVRNSKRGAAGSLMNVLDHPGMGHRVEITEGILADECAALLCDFYCMPRQVFNAQKKAQSSISSGGSSGGSSGSDTPGTRESATPESSGGGSSGSAKNTITKALQLRIVRPYNSAEVEKIVADEKNNREKIALEKNKDKVREACSKHLKVASYCTTQVERNACPFCKARKLDDKFYQKLRGQFPDAVFWQELGEIFRQLQKQAAEVYNQSLIELYYEIFIKGKGFANASSVEHYLSDVCYTRAAELFKNAAIASGLRGKVKSNFRLKELKNMKSGLPTTKSDNFPIPLVKQKGGQYTGFEISSHNDDLVIKIPFGRWRVKREIDKYRPWEKFDFEQVRKSPKPISLLLSTQRRKRNKGWSEDEGTEAEIRKMMNGDYQTSYIEVKRGSKIGEKSAWMLNLSIDVPKIDKGVDPSIIGGIDVGVKSPLVCAINNAFSRYSIGDNDLFHYNKKMFARRRILLKKNRHKRAGHGAKNKLRPISILTEKSKRFRKKLIERWACEIADFFIKNKVGTVQMENLESMKRKEDSYFNIRLRGFWPYAEMQNKIEFKLKQYGIEIRKVAPNNTSKTCSKCGHLNNYFNFEYRRKSKFPHFKCEKCNFKEDADYNAALNISNPKLKSTKEEP

SEQ ID NO: 2648 - protein, 726 aa, synthetic construct
SEVEFSHEYWMRHALTLAKRARDEREVPVGAILVLNNRIIGEGWNRAIGLHDPTAHAEIMALRQGGLVMQNYRLIDATLYVTFEPCVMCAGAMIHSRIGRVVFGARNSKHGAAGSLVNVLNYPGMNHRVEITEGILADECAALLCDFYRMPRRVFNARMKAQSSISPGGPSGGSSGSETPDTSESATPESSGGNSGSSAKNTITKTLKLRIVRPYNSAEVEKIVADEKNNREKIALEKNKDKVKEACSEHLKVAAYCTTQVERNACLFCKARKLDDKFYQKLRGQFPEAVFWQEIGEIFRQLQKQAAEIYNQSLIELYYEIFIKGKSIANASSVEHYLSDVCYTKAAELFRNAAIASGLRSKIKSNFRLKELRNMKSGLPTTKSDNFPIPLVKQKGGQYTGFEISNHNSDFIIKIPFGRWQVKKEIDKYRPWEKFDFEQVRKSPKPISLLLSTQRRKRNKGWSKDEGTEAEIKKVMNGDYQTSYIEVTRGSKIGEKSAWMLNLSIDVPKIDKGVDPSIIGGIDVGVKSPLVCAINNAFSRYSISDNDLFHFNKKVFARRRILLKKNRHKRAGHGAKNKLKPITILTGKSKRFRKKLIERWACEIADFFVKNKVGTVQMENLESMKRKEDSYFNIRLRGFWPYAEMQNKIEFKLKQYGIEIRKVAPNNTSKTCSKCGHLNNYFNFEYRKKNKFPHFKCEKCNFKENADYNAALNISNPKLKSTKGEP

SEQ ID NO: 2649 - protein, 726 aa, synthetic construct
SEVEFSHEHWMRHALTLAKRARDEREVPVGAVLVLNNRVIGEGWNRAIGLHDPTAHAEIMALRQGGLVMQNYRLIDATLYVTFEPCIMCAGAMIHSRIGRVVFGVRNSKRGAAGSLMNVLNYPGMNHRVEITEGVLADECAALLCDFYRMPRQVFNARKKAQPSINPGGSSGGSSGSETPGTSESATPESSGGSSGGSAKNTITKTLKLRIVRPYNSAEVEKIVADEKNNREKIALEKNKDKVKEACSKHLKVAAYCTTQVERSACLFCKARRLDDKFYQKLRGQFPDAVFWQEIGEIFRQLQKQAAETYNQSLIELYYEIFIKGRGFANASSVEHYLSDVCYTRAAELFKNAAIASGLRGKVKSNFRLKELKNMRSGLPTTKSDNFPIPLVKQKGGQYTGFEISNHNSDFIIKIPFGRWQVKKEINKYRPWEKFDFEQVRKSPKPISLLLSTQRRKRNRGWSKDEGTEAEVKKVMNGDYQISYIEVKRGSKIGEKSAWMLNLSIDVPKIDKGVDPSIIGGIDVGVKSPLVCAISNAFSRYSISDNDLFHFNKKMFARRRILLKKSKHKRAGHGAKNKLKPITILTEKSRRFRKKLIERWACEIADFFIKNKVGTVQMENLESMKRKEDSYFNIRLRGFWPYAEMQNKIEFKLKQYGIEIRKVAPNNTSKTCSKCGHLNNYFNFEYRKKNKFPRFKCEKCNFKENADYNAALNISNPKLMSTKEEP

SEQ ID NO: 2650 - protein, 726 aa, synthetic construct
SEVEFSHEYWMRHALTLAKRARDEREVPVGAVLVLNNRAIGEGWNRAIGLHDPTAHAEIMALRQGGLVMQNCRLTDATLYVTFEPCVMCAGAMVHSRIGRVVFGVRNSKRGAAGSLMNVLNYPGVNHCVEITEGILVDECAALLCDFYRMPRQVFNARKKAQSSINPGGSSGGSSGSETPGASGSVTPKSSGGSSAGSTKDTITKTLKLRIVRPYNSAEVEKVVADEKNNREKIAIEKNKDMVKEACSKHLKVASYCTTQVERNACLFCKARKLDDKFYQRLRGQFPDAVFWQELGEIFRQLQKQAAEIYNQSLIELYYEIFIKGKGFANASSVEHYLSDVCYTRAAELFKNAAIASGLRGKVKSNFRLKELKNMKSGLPTTKSDNFPIPLVRQKGGQYTGFEISSHNDDFIIKIPFGRWQVRKEIDKYRPWEKFDFEQVRKSPKPISLLLSTQRRKRNKGWSKDEGTEAEIRKVMSGDYQTSYIEVKRGSKIGEKSAWMLNLSIDVPKIDKGVDPSIVGGIDVGVKSPLVCAINNALGRYSISDNDLFHFNKKMFARRRILLKKNGRKRAGHGARNKLKPITALTEKSKRFRKKLIERWACEIANFFIKNRVGTVQMENLESMKRKEDSYFNIRLRGFWPYAEMQNRIEFKLKQYGIEIRKVAPNNTSKTCSKCGHLNNYFNFEYRKKNKFPHFRCEKCNFKEDADYNAALNICNPKLKGTKEEP

SEQ ID NO: 2651 - protein, 726 aa, synthetic construct
SEVEFSHEYWMRHALTLAKRARDEREVPVGAILVLNNRVIGEGWNRAIGLHDPTAHAEIMALRQGGLVMQNYRLVDATLYVTFEPCVLCAGAMVHSRIGRVVFGVRNSKRGAAGSLMNVLNYPGMNHRVEVTEGILADECAALLCDFYRMPRQVFNARKKARSNINSGGSSGGSSDSETPGTSESATPESSGGSSGSSAKNTITKTLKLRIVRPYNSAEVEKIVADEKNNREKIALEKNKDKVKEACSKHLKVAAYCTTQVERNACLFCKARRLDDKFYQKLRGQFPDAVFWQEIGEIFRQLQKQAAEVYNQSLVELYYEILIKGKGIANASSVEHYLSDVCYTRAAELFKNAAIASGLRNKIKSNFRLKELRNMKSGLPTTKSDNFPIPLVRQKGGQYTGFEISNHDGDFIIKIPFGRWQVKKEIDKYRPWEKFDFEQVRKSPKPISLLLSTRRRKRNKGWSKDEGTGAEIRKVMNGDYQTSYIEVKRGSKIGEKSAWMLNLSIDVPKIDKGVDPSIIGGIDVGVKSPLVCAINNAFGRYSISDNDLFHFNKKMFARRRILLKKNRHRRAGHGARNKLKPITVLTEKSKRFRKKLIERWACEIANFFVKNKVGTVQMENLESMKRKEDSYFNIRLRGLWPYAEMQNKIEFKLKQYGIEVRKVAPNNTSKTCSKCGHLNNYFNFEYRKRNKFPHFKCEKCNFKENADYNAALNISNPKLKATKEEP

SEQ ID NO: 2652 - protein, 726 aa, synthetic construct
SEDEFSHEYWMRHALTLAKRARDGREVPVGAVLVLNNRVIGEGWNRAIGLHDPTAHAEIMALRQGGLVMQNYRLIDATLYVTFEPCVMCAGAMVHSRIGRVVFGVRNSKRGAAGSLMNVLDYPGMNHRVEITEGILADECAALLCDFYRMPRQVFNARKKAQSSINPSGSSGGSSGSETPGTSESVAPESSGGSSGGSAKNTITKTLKLRIVRPYNSAEVEKIVADEKNNREKIALEKNKDKVKEACSKHLKVAAYCTTQVERNACLFCRARRLDDEFYQKLRGQFPDAVFWQEIGEIFRQLQKQAAEIYNQSLIELYYEIFIKGKGFANASSVEHYLSDVCYTRAAELFKNAAIASGLRGKVKSNFRLKELKNMKSGLPTTKSDNFPIPLVRQKGGQYTGFEISSHNDDFIIKIPFGRWQVRKEIDKYRPWEKFDFEQVRKSPKPISLLLSTQRRKRNKGWSKDEGTEAEIRKVMSGDYQTSYIEVKRGSRTGEKSAWMLNLSIDVPKIDKGVDPSVIGGIDVGVKSPLVCAINNAFSRFSISDNDLFHFNKKMFARRRILLKKNGRKRAGHGAKNKLKPITILTEKSKRFRKKLIERWACEIAGFFIKNKVGTVQMENLESMKRKEDSYFNIRLRGFWPYAEMQNKIEFKLRQYGIVVRKVAPNNTSKTCSQCGHLNNYFNFEYRKKNKFPYFKCEKCNFKENADYNAALNISNPQLKSTKGEP

SEQ ID NO: 2653 - protein, 726 aa, synthetic construct
SEVEFSHEYWMRHALTLAKRARDEREVPVGAILVLNNRVIGEGWNRAIGLHDPTAHAEIMALRQGGLVMQNYRLIDATLYVTFEPCVMCAGAMIHSRIGRVVFGVRNSKHGAAGSLVNVLNYPGMNHRVEITEGILADECAALLCDFYRMPRQVFNARKKAQSSINSGGSSGGSSGSETPGTSESATPKSSGGSSGGSAKNTITKALKLRIVRPYNSAEVEKIVADEKNNRERIALERNKDKVKEACSKHLKVAAYCTTQVERNACLFCKARKLDDKFYQKLRGQFPDAVFWQETGEIFRQLQRQAAEIYNQSLIELYYEIFIKGKGFANASSVEHYLSDVCYTRAAELFKNAAIASGLRGKVKGNFRLKELKNMKSGLPTTKSDNFPIPLVKQKGGQYTGFEISSHNDDFIIKIPFGRWQAKKEIDKYRPWEKFDFEQVRKSPKPISLLLSTQRRKRNKGWSKDEGTEAEIRKVMNGDYQTSYIEVKRGSKIGEKSAWMLSLSIDVPKIDKGVDPSIIGGVDVGVKSPLVCAINNAFSRYSISDNDLFRFNKKMFARRRILLGKNRHKRAGHGVKNKLKPITILTEKSGRFRKKLIERWACEIADFFIKNKVGTVQMENLESMKRKEDSYFNIRLRGFWPYAEMQNKIEFKLKQYGIKIRKVAPNNTSKTCSKCGHLNNYFSFEYRKKNKFPRFKCEKCNFKENADYNAALNISNPKLMSTKEEP

SEQ ID NO: 2654 - protein, 726 aa, synthetic construct
SEVEFSHEYWMRHALTLAKRARDEREVPVGAVLVLNNRVIGEGWNRAIGLHDPTAHAEIMALRQGGLVMQNYRLTDATLYVTFEPCVMCAGAMIHSRIGRVVFGVRNGKRGAAGSLMNVLNYPGMNHCVEITEGILVDECAALLCDFYRMPRQVLNAQKKAQSSISSGGSSGGSNGSETPGASESATPKSSDGSSAGSTKNTITKTLKLRIVRPYNSAEVEKIVADEKNSREKTALEKNKDKVKEACSKHLKVAAYCTTQVERSACLFCRARKLDDKFYQKLRGQFPDAVFWQELGEIFRQLQKQAAEIYNQSLIELYYEIFIKGKGFANASSVEHYLSDVCYTRAAELFKNAAIASGLRGKVKSNFRLKELKNMKSGLPTTKSDNFPIPLVKQKGGQYTGFEISSHNDDFIIKIPFGRWQVRKEIDKYRPWEKFNFEQVRKGPKPISLLLSTQRRKRNKGWSKDEGTEAEIRKVMNGDYQTSYIEVKRGSKIGEKSAWMLSLSIDVPKIDKGVDPNIVGGIDVGVKSPLVCAINNALGRFSISDNDLFHFNKKMFARRRILLRKNRHKRAGHGAKNKLKPISILTEKGKRFRKKLIERWACEIADFFIKNKVGTVQMENLESMKRKEDSYFNIRLRGFWPYAEMQNKIELKLKQYGIKIRKVAPNNTSKTCSKCGHLNDYFNFEYRKRNKFPHFKCEECNFKEDADYNAALNISNPKLKSTREEP

SEQ ID NO: 2655 - protein, 726 aa, synthetic construct; identical to SEQ ID NO: 684

SEQ ID NO: 2656 - protein, 726 aa, synthetic construct
SEVEFSHEYWMRHALTLAKRARDEREVPVGAVLVLNNRVIGVGWNRAIGLHDPTAHAEIMALRQGGLVTQNYRLVDATLYVTFEPCVMCAGAMIHSRIGRVVFGVRNGKRGAAGSLMNVLNYPGMNHRVEITEGILVDECAALLCDFYRMPRRVFNAQKKAQSNINPGGSSGGSSGSETPGTSESPTPESSRGSPGGSAKNTITKTLKLRIVRPYNSAEVEKIVAEEKDNREKIALEKNKDKVREACSKHLKVAAYCTTQVERNACLFCKARKLDDKFYQKLRGQFPDAVFWQEIGEIFRQLQKQAAEIYNQSLIELYYEIFIKGKGFANASSVEHYLSDVCYTRAAELFKNAAIASGLRGKVKSNFRLKELKNMKSGLPTTKSDNFPIPLVKQKGGQYTGFEISSHNDDFIIKIPFGRWQAKKEIDKYRPWEKFDFEQVRKSPKPISLLLSTQRRKRNKGWSKDEGTEAEIKKVMNGDYQTSYIEVKRGSKIGEKSAWMLNLSIDVPKIDKGVDPRIIGGIDVGVRSPLVCAINNAFSRYSISDNDLFHFNKKMFARRRILLKKNRHKRAGHGATNKLKPITIPTEKSERFRKKLIERWACEIADFFVKNKVGTVQMENLESMKGKEDSYFNIRLRGFWPYAEMQNKIEFKLKQYGIKIRKVAPNNTSKTCSKCGHLNNYFSFEYRKKNKFPHFKCEKCNFKEDADYNAALNISNPKLKSTKEEP

SEQ ID NO: 2657 - protein, 726 aa, synthetic construct
SEVEFSHEYWMRHALTLAKRARDEREVPVGAVLVLNNRVIGEGWNRTTGQHDPTAHAEIMALRQGGLVMQNHRLVDATLYVTFEPCVMCAGAMIHSRIGRVVFGVRNSKRGAAGSLTNVLNYPGMNHRVEITEGILVDECAALLCDFYRMPRRVFNAQKRAQSTINTGGSTGGSSGSETPGTSESPTPESSGGSPGGSAKNTITKTLKLRIVRPHNSAEVEKIVADEKNNREKIALEKNKDKVKEACSKHLKVAAYCTTQVERNACLFCRARKLDDKFYQKLRGQFPDAVFWQEIGEIFRQLQKQAAEIYNQSLIELYYEIFIKGKGFANASSVEHYLSDVCYTRAAELFKNAAIASGLRGKVRSNFRLKELKSMKSGLPTTKSDNFPIPLVKQKGGQYTGFEISSHNDDFIIKIPFGRWQVKEEIDKYRPWEKFDFEQVRKNPKPISLLLSTLRRKRNKGWSKDEGTEAEIRKVMNGDYQTSYIEVKRGSKIGEKSAWMLNLSIDVPKIDKGADPSIIGGIDVGVKSPLVCAINNAFSRYSISDNDLFRFNKKVFARRRILLKKNRHKRAGHGTKNKLKPITILTEKSGRFRKKLIERWACEIANFFIKNKVGTVQMENLESMKRKEDSYFNIRLRGFWPYAEMQNKIEFKLKQYGIKIRKVAPNNTSKTCSKCGHLNNYFSFEYRRKNKFPHFKCEKCNFKEDADYNAALNISNPKLKSTKEEP

SEQ ID NO: 2658 - protein, 726 aa, synthetic construct
SEVEFSHEYWMRHALTLAKRARDEREVPVGAVLVLNNRVIGEGWNRAIGLHDPTAHAEIMALHQGGLVMQNYRLIDATLYVTFEPCVMCAGAMIHSRIGRVVFGARNSKRGAAGSLMNVLSYPGMNHRVEITEGILADECAALLCDFYHMPRRVFNAQKKAQSSINSGGSSGGGSGSETPSTSESTTPESSGGSSGGPAKNTITKTLKLRIVRPYNSAEVEKIVADEKNNREKTALEKNKDKVKEACSKHLKVAAYCTTQVERNACLFCKARKLDDKFYQKLRGQYPDAVFWQEVGEIFRQLQKQAAEIYNQSLIELYYEIFIKGKGFANASSVEHYLSDVCYTRAAELFKNAAIASGLRNKIKSNFRLKELRNMKSGLPTTKSDNFPIPLVRQKGGQYTGFEISNHDGDFIIKIPFGRWQVKKEINKHRPWEKFDFEQVRKSPKPISLLLSTQRRKRNKGWSKDEGTEAEIRKVMNGDYQTSYIEVKRGSKIGEKSAWMLNLSIDVPKIDKGVDPSIIGGIDVGVKSPLVCAINNALSRYSISDNDLFHFNKKMFARRRILLKKNRHKRAGHGAKNKLKPITVLTEKSERFRKKLIERWACEIANFFIKNKVGTVQMENLESMKRREDSYFNIRLRGFWPYAEMQSKIEFKLKQYGIKIRKVAPNNTSKTCSKCGHLNNYFNFEFRKKNKFPHFKCEKCNFKEDADYNAALNISNPKLKSTKEEP

SEQ ID NO: 2659 - protein, 726 aa, synthetic construct
SEVEFSHEYWMRHALTLAKRARDEREVPVGAILVLNNRVIGEGWNRAIGLHDPTAHAEIMALRQGGLVMQNYRLIDATLYVTFEPCVMCAGAMIHSRIGRVVFGVRNNKHGAAGSLVNVLNYPGMNHRVEITEGILADECAALLCDFYCMPRQVFNAQRRAQSSINPGGSSGGSSGSETPGTSESASPESSGGGSSGSAKNTITKTLQLRIVRPYNSAEVEKIVADEKNNREKIALEKNKDKVKEACSKHLKVASYCTTQVERNACPFCKARKLDDKFYQKLRGQFPDAVFWQELGEILRQLQKQAAEIYNQSLIELYYEIFIKGRGFANACSVEHYLSDVCYTRAAELFKNAAIASGLRGKVKSNFRLKELKNMKSGLPTTKSDNFPIPLVKQKGGQYTGFEISSHNDDLIIKIPFGRWQVKKEIDKYRPWEKFDFEQVRKSPKPISLLLSTQRRKRNKGWSKDEGTEAEIRKVMNGDYQTSYIEVRRGSKTGEKSAWMLNLSIDVPKIDKGVDPSIIGGIDVGVKSPLVCAINNALSRYSISDNDLFRFNKRMFARRRILLRGNRHKRAGHGAKNKLKPITILTEKSKRFRKKLIERWACEIADFFIKNKVGTVQMENLESMKRKEDSYFNIRLRGLWPYAEMQNKIEFKLKQYGIEIRKVAPNNTSKTCSKCGHLNNYFNFEYRKRNKFPHFKCEKCNFKENADYNAALNISNPKLKSTKGEP

SEQ ID NO: 2660 - protein, 726 aa, synthetic construct
SEVKFSHEYWMRHALTLAKRARDEREVPVGAILVLNNRVIGEGWNRAIGLHDPTAHAEIMALRQGGLVMQNYRLIDATLYVTFEPCVMCAGAMIHSRIGRVVFGVRNSKHGAAGSLVNVLNYPGMNHRVEITEGILADECAALLCDFYRMPRRVFNARKKAQSSIDPGGPSGGSSGNETPGTSESATPESSGGSSGGSAKNTITKTLKLRIVRPYNSTEVEKIVADEKNNREKVALEKNKDKVKEACSKHLKVASYCTTQVERNACLFCKARKLDDKFYQKLRGQFPDAVFWQEIGEIFRQLQKQAAEIYNQSLIELYYEIFIKGKGFANASSVEHYLSDVCYTRAAELFKNAAIASGLRGKVKSNFRLKELKNMKSGLPTTKSDNFPIPLVKQKGGQYTGFEISSHSDDFIIKIPFGRWQVKKEIDKYRPWEKFDFEQVRKSPKPISLLLSTQRRKKNKGWSKDEGTEAEIRRVMNGDYQTSYIEVKRGSKIGEKSAWMLNLSIDVPKIDKGVDPSIIGGIDVGVKSPLVCAINNSSSRYSICDNDLFRFNKKMFARRRILLKKNRHKRAGHGAKNKLKPITILTKKSERFRKKLIERWVCEVADFFIKNKVGTVQMENLESMKRKEDSYFNIRLRGFWPYAEMQNRIELKLKQYGIEIRRVAPNNTSRTCSKCGHLNNYFSFEYRKKNKFPHFKCEKCNFKEDADYNAALNISNPKLKGTKEEL

SEQ ID NO: 2661 - protein, 726 aa, synthetic construct
SEVEFSHEYWMRHALTLAKRARDEREVPVGAILVLNNRVIGEGWNRAIGLHDPTAHAEIMALRQGGLVMQNYRLIDATLYVTFEPCVMCAGAMIHSRIGRVVFGVRNSKHGAAGSLVNVLNYPGVNHCVEITEGILADECAALLCDFYRMPRQVFNAQKKAQSSINSGGPSGGSSGSETPGASESATPESSGGSSGGSAKNTITKTLQLRIVRPYNSAEVEKIVTDEKNNREKIALEKNKDKVKEACSKHLKMASYCTTQVERNACLFCKARKLDDKFYQKLRGQFPDAVFWQELGEIFRQLQKQAAEIYNQSLVELYYEILIKGKGIANASSVEHYLSGVCYTRAAELFKNAAIASGLRNKIKSNFRLKELRNMKSGLPTTKSDNFPIPLVKQKGGQYTGFEISSHNDDFIIKIPFGRWQVKEEIDKYRPWEKFDFEQVRKNPKPISLLLSTRRRKRNKGWSKDEGTEAEIRKVMNGDYQTSYIEVKRGSKTGEKSAWMLNLSIDVPKIDKGVDPSIIGGIDVGVKSPLVCAINNAFSRYSISDNDLFRFNKKMFARRRVLLKKNRHKRAGHGAKNKLKPISILTRKGERFRKKLIERWACEIADFFIKNKVGTVQMENLESMKRKEDSYFNIRLRGFWPYAEMQNKIEFKLKQYGIEIRKVAPNNTSKTCSKCGHLNSYFNFEYRKKNKFPHFKCEKCNFKENADYNAALNISNPKLKSTKEEP

SEQ ID NO: 2662 - protein, 726 aa, synthetic construct
SEVEFSHEYWMRHALTLAKRARDEREVPVGAVLVLNNRVIGEGWNRTTGLHDPTAHAEIMALRQGGLVMQNHRLVDATLYVTFEPCVMCAGAMIHSRIGRVVFGVRNSKRGAAGSLTNVLNYPGMNHRVEITEGILVDECAALLCDFYRMPRQVFNARKKAQSSINPGGSSGGSSGSETPGTSESATPESSGGSSGSSAKNTITKTLKLRIVRPYNSAEVEKIVADEKNNREKVALEKNKDKVKEACSKHLKVAAYCTTQVERNACLFCKARKLDDKFYQKLRGQFPDAVFWQEIGEILRQLQKQAAEVYNQSLIELYYEIFVKGKGFANASSVEHYLSDVCYTRAAELFKNAAIASGLRGKVKSNFRLKELKNMKSGLPTTKSDNFPIPLVKQKGGQYTGFEISSHNDDFIIKIPFGRWQVKEEIDRYRPWEKFDFEQVRKSPKPISLLLSTQRRKRNKGWSKDEGTEAEIRKVMNGDYQTSYIEVRRGSKIGERSAWMLNLSIDVPKIDKGVNPSIIGGIDVGVRSPLVCAINNAFSRYSISDNDLFRFNKRMFARRRILLGKNRHKRAGHGVKNKLKPITILTEKSGRFRKKLIERWACEIADFFVKNKVGTVQMENLESMKRKEDSYFNIRLRGFWPYAEMQNKIEFKLKQYGIKVRKVAPNNTSKTCSKCGHLNNYFSFEYRKKNKFPHFKCEKCNFKENADYNAALNISNPKLKSTKEEP

SEQ ID NO: 2663 - protein, 726 aa, synthetic construct
SEDEFSHEYWMRHALTLAKRARDGREVPVGAVLVLNNRVIGEGWNRAIGLHDPTAHAEIMALRQGGLVMQNYRLIDATLYVTFEPCVMCAGAMVHSRIGRVVFGVRNSKRGAAGSLMNVLNYPGMGHRVEITEGILADECAALLCDFYCMPRQVFNAQKRAQFSINSGGSSGGSSGSETPGSSESATPESSGGGSSGSAKNTITKALQLRIVRPYNSAEVEKIVADEKNNREKIALEKNKDKVKEACSKHLKVASYCTTQVERNACPFCKARKLDDKFYQKLRGQFPDAVFWQELGEILRQLQKQAAEIYNQSLIELYYEIFIKGRGFANAGSVEHYLSDVCYTRAAELFKNAAIASGLRGKVKSNFRLKELKNMKSGLPTTKSDNFPIPLVKQKGGQYTGFEISSHNDDFIIKIPFGRWQVKKEIDKYRPWEKFDFEQVRKSPKPISLLLSTQRRKRNKGWSKDEGTEAEIRKVMNGDYQTSYIEVKRGSKTGEKSAWMLNLSIDVPKIDKGVDPSIIGGIDVGVKSPLVCAINNAFSRYSISDNDLFRFNKKMFARRRILLKKNRHKRAGHGAKNKLKPISILTGKSERFRKKLIERWACEIADFFIKNKVGTVQMENLESMKRKEDSYFNIRLRGFWPYAEMQNKIEFKLKQYGIEIRRVVPNNTSKTCSKCGHLNNYFNFEYRKKNKFPHFKCEKCNFKENADYNAALNISNPELKSTKEEP

SEQ ID NO: 2664 - protein, 726 aa, synthetic construct
SEVEFSHEYWMRHALTLARRARDEREVPVGAILVLNNRVIGEGWNRAIGLHDPTAHAEIMALRQGGLVMQSYRLVDATLYVTFEPCVMCAGAMIHSRIGRVVFGVRNSKHGAAGSLMNVLNYPGMNHRVEITEGILADECAALLCDFYCMPRQVFNAQKRAQSSINSGGSSGGSSGSETPGTSESATPEGSGGGSSGSAKNTITKTLQLRIVRPYNSAEVEKIVADEKNNREKIALEKNKDKVKEACSKHLKVASYCTTQVERNACLFCKARKLDDKFYQKLRGQFPDAVFWQELGGIFRQLQKQAAEIYNQSLIELYYEIFIKGKGITNASRVEHYLSDVCYARAAELFKNAAIASGLRSKVRSNFRLKELKNMKSGLPTTKSDNFPIPLVKQKGGQYTGFEISSHNDDFIIKIPFGRWHVKKEIDKYRPWEKFDFGQVRRSPKPISLLLSTQRRKRNKGWSKDEGTEAEIRKVMNGDYQTSYIEVKRGSKIGEKSAWMLSLSIDVPKIDKGVDPSIIGGIDVGVKSPLVCAINNAFCRYSISDNDLFHFNKKMFARRRILLKRSRHKRAGHGAKNKLKPISILTEKSKRFRKKLIERWACEIADFFIKNKVGTVQMENLESMKRKEDSYFNIRLRGFWPYAEMQNKIEFKLKQYGIEIRKVAPNNTSKTCSKCGHLNNYFNFEYRKKNKFPHFKCEKCNFKENADYNAALNISNPKLKSTKEEP

SEQ ID NO: 2665 - protein, 726 aa, synthetic construct
NEVEFSHEYWMRHALTLAKRARDEREVPVGAVLVLNNRVIGEGWNRTTGLHDPTAHAEIMALRQGGLVMQNHRLVDATLYVTFEPCVMCAGAMIHSRIGRVVFGVRNSKHGAAGSLVNVLDYPGMNHRVEITEGILADECAALLCDFYRMPRQVFNARKKAQSSISPGGSSGGSSGSETPGTSESATPKSSGGSSGGSAKNTITKTLKLRIVRPYNSAEVEKIVADEKNNREKIALEKNKGKVKEACSKHLEVAAYCTTQVERNACLFCKARKLDDKFYQKLRGQFPDAVFWQELGEIFRQLQKQAAEIYNQSLIELYYEIFIKGKGFANASGVEHYLSDVCYTRAAELFKNAAIASGLRGKVKSNFRLKELKNMKSGLPTTKSDNFPIPLVKQKGGQYTGFEISSHNDDFIIKIPFGRWQVKKEIDRYRPWEKFDFEQVRKSPKPISLLLSTQRRKRNKGWSKDEGTEAEIRKVMNGDYQTSYIEVKRGSKTGEKSAWMLNLSIDVPKIDKGVDPSIIGGIDVGVKSPLVCAINNAFSRYSVSDNDLFRFNKKMFARRRILLKKNRHKRAGHGAKNKLKPISILTGKSERFRKKLIERWACEIADFFIKNKVGTVQMENLESMKRKEDSYFNIRLRGLWPYAEMQNKIEFKLKQYGIEVRKVAPNNTSKTCSKCGHRNNYFNFEYRKRNKFPHFKCEKCNFKENADYNAALNISNPKLKGTKEEP

SEQ ID NO: 2666 - protein, 726 aa, synthetic construct
SEDEFSHEYWMRHALTLAKRARDEREVPVGAVLVLNNRVIGEGWNRAIGLHDPTAHAEIMALRQGGLVMQNYRLIDATLYVTFEPCVMCAGAMVHSRIGRVVFGVRNSKRGAAGSLMNVLDYPGMGHRVEITEGILADECAALLCDFYCMPRQVFNAQKRAQSSINSGGSSGGSSGSETPGTSESATPESSGGGSSGSAKNTITKALQLRIVRPYNSAEVEKIVADEKNNREKIALEKNKDKVKEACSKHLKVAPYCTTQVERNACPFCKARKLDDKFYQKLRGQFPDAVFWQELGEILRQLQKQAAEIYNQSLIELYYEIFIKGRGFANASSVEHYLSDVCYTRAAELFKNAAIASGLRGKVKSNFRLKELKNMKSGLPTTKSDNFPIPLVKQKGGQYTGFEISSHDDDFIIKIPFGRWQVKEEIDKYRPWEKFDFEQVRKSPKPISLLLSTQRRKKNKGWSKDEGTEAEIRRVMNGDYQTSYIEVKRGSKTGEKSAWVLNLSIDVPKIDKGVDPSIIGGIDVGVKSPLVCAINNAFSRYSISDNDLFRFNKKMFARRRILLKKNRHKRAGHGAKNKLKPIAVLAEKSEGFRKKLIERWACEIADFFIKNKVGTVQMENLEGMKRKEDSYFNIRLRGFWPYAEMQNKIEFKLKQYGIEVRKVAPNNTSKTCSKCGHLNNYFNFEYRRKNKFPHFKCEKCNFKENADYNAALNISNPKLKSTKEEP

SEQ ID NO: 2667 - protein, 726 aa, synthetic construct
SEVEFSHEYWMRHAMSLAKRARDEREVPVGAVLVLNNRVIGEGWNRAIGLHDPTAHAEIMALRQGGLVMQNYRLSDATLYVTFEPCVMCAGAMIHSRIGRVVFGVRNSKRGAAGSLMNVLNYPGMNHCVEITEGILVDECAALLCDFYRMPRQVLNAQKKAQSSISPGGSSGGSSGSETPGASESVTPKSSGGSSGGSAKDTITKTLKLRIVRPYNSAEVEKIVTDEKNNREKIALEKNKDKVKEACSKHLKMASYCTTQVERNACLFCKARKLDDKFYQKLRGQFPDAVFWQELGGIFRQLQKQAAEIYNQSLIELYYEIFIKGKGITNASRVEHYLSDVCYTRAAELFKNAAIASGLRSKVRSNFRLKELKNMKSGLPTTKSDNFPIPLVKQKGGQYTGFEISSHNDDFIIKIPFGRWQVRKEINKHRPWEKFDFEQVRKSPKPISLLLSTQRRKRNKGWSKDEGTEAEIRKVTNGDYQTSYIEVKRGSKIGEKSAWMLNLSIDVPKIDKGVDPSIIGGIDVGVKSPLVCAINNALSRYSISDNDLFHFNKRMFARRRILLRKNRHKRAGHGAKNKLKPITIMTEKSKRFRKKLIERWACEIADFFIKNKVGTVQMENLESMKRREDSYFNIRLRGFWPYAEMQNKIEFKLKQYGIVVRKVAPNNTSKTCSKCGHLNSYFNFEYRKRNKFPHFKCEKCNFKEDADYNAALNISNPKLKSTKGEP

SEQ ID NO: 2668 - protein, 726 aa, synthetic construct
SEDEFSHEYWMRHALTLAKRARDGREVPVGAVLVLNNRVIGEGWNRAIGLHDPTAHAEIMALRQGGLVMQNYRLIDATLYVTFEPCVMCAGAMVHSRIGRVVFGVRNSKRGAAGSLMNVLDYPGMGHRVEITKGILADECAALLCDFYCMPRQVFNARKKAQSSINSGGSSDGGSGSETPGTSESATPESSGGSSGGSAKNTITKTLKLRIVRPYNSAEVEKIVADEKNNREKIALEKNKDKVKEACSEHLKVAAYCTTQVERSACLFCKARKLDDKFYQKLRGQFPDAVFWQEIGEIFRQLQKQAAEIYNQSLIELYYEIFIKGKGFANASSVEHYLSDVCYTRAAELFKNAAIASGLRGKVKSNFRLKELKNMKSGLPTTKSDNFPIPLVKQKGGQYTGFEISSHNDDFIIKIPFGRWQVKEETDKYRPWEKFDFEQVRKSPKPISLLLSTQRRKRNRGWSKDEGTEAEIRKVMNGDYQTSYIEVKRGSRFGEKSAWMLNLSIDVPKIDKGVDPSIIGGIDVGVKSPLVCAINNAFSRYSISDNDLFRFNKKMFARRRILLGKNRLKRAGHGVKNKLKPITILTEKSGRFRKKLIERWACEIADFFVKNKVGTVQMENLESMKRKEDSYFNIRLRGFWPYAEMQNKIEFKLKQYGIKVRKVAPNNTSKTCSKCGHLNNYFSFEYRKKNKFPHFKCEKCNFKENADYNAALNISNPKLKSTKEEP

SEQ ID NO: 2669 - protein, 726 aa, synthetic construct
SEVEFSHEYWMRHALTLAKRARDEREVPVGAVLVLNNRVIGEGWNRTTGLHDPTAHAEIMALRQGGLVMRNYRLTDATLYVTFEPCVMCAGAMIHSRIGRVVFGVRNSKRGAAGSLMNVLNYPGMNHCVEITEGILVDECAALLCDFYRMPRQVLSAQKKAQSSVSSGGSSGGSSGSETPGASGSVTPKSSVGSSAGSTKNTITKTLKLRIVRPYNSAEVEKIVADEKNNREKIALEKNRDKVKEACSKHLKVAAYCTTQVERNACLFCKARKLDDKFYQKLRGQFPDAVFWQELGGIFRQLQKQAAEIYNQSLIELYYEIFIKGKGITNASRVEHYLSDVCYTRAAELFKNAAIASGLRSKVKSNFKLKELKSMKSGLPSTKSDNFPIPLVKQRGGQYTGFEISNHNGDFIIKIPFGRWRVKREINKYRPWEKFDFEQVRKSPKPISLLLSTQRRKRNKGWSKDEGTEAEIRKVMNGDYQTSYIEVKRGSRIGEKSAWMLSLSIDVPKIDRGVDPSIIGGIDVGVKSPLVCAINNALSRYSISDNDLFHFNKKMFARRRILLKKNRHRRAGHGARNKLKPITVLTEKSKRFRKKLIERWACEIANFFVKNKVGTVQMENLESMKRKEDSYFNIRLRGLWPYAEMQNKIEFKLKQYGIEVRKVAPNNTSKTCSKCGHLNNYFNFEYRKKNKFPHFKCEKCNFKENADYNAALNISNPKLKSTKEEP

SEQ ID NO: 2670 - protein, 726 aa, synthetic construct
SEVEFSHEYWMRRALTLAKRARDEREVPVGAILVLNNRVIGEGWNRAIGLHDPTAHAEIMALRQGGLVMQNHRLIDATLYVTFEPCVMCAGAMIHSRIGRVVFGVRNSKHGAAGSLVNVLNYPGMNHRVGITEGILADECAALLCDFYRMPRQVFNAQRRARSSINSGGSSDGSSGSETPGTSESATPESSGGGSSGSAKNTITKTLQLRIVRPYNSAEVEKIVADEKNNREKIALEKNKDKVREACNKHLKVASYCTTQVERNACPFCKARKLDDKFYQKLRGQFPDAVFWQELGEILRQLQKQAAEIYNQSLIELYYEIFIKGKGFANASSVEHYLSDVCYTRAAELFKNAAIASGLRGKVKGNFRLKELKNMKSGLPTTKSDNFPIPLVKQKGGQYTGFEISSHNDDFIIKIPFGRWQAKKEIDKYRPWEKFDFEQVRKSPKPISLLLSTQRRKKNKGWSKDEGTEAEIRRVMNGDYQTSYIEVMRGSKIGEKSAWMLSLSIDVPKIDKGVDPSIIGGIDVGVKSPLVCAINNAFNRYSISDNNLFHFNKKMFARRRILLKKNRHKRAGHGAKNKLKPISILTEKSERFRKKLIERWACEIADFFIRNKVGTVQMENLEGMKRREDSYFNIRLRGFWPYAEMQNKIEFKLKQYGIEVRKVAPNNTSKTCSKCGHLNNYFNFEYRKKNKFPHFKCEKCNFKENADYNAALNISNPKLKSTKEEP

SEQ ID NO: 2671 - protein, 726 aa, synthetic construct
SEVEFSHEYWMRHALTLAKRARDEREVPVGAILVLNNRVIGEGWNRAIGLHDPTAHAEIMALRQGGLVMQNYRLTDATLYVTFEPCVMCAGAMIHSRIGRVVFGVRNSKHGAAGSLVNVLNYPGMNHRVEITEGILADECAALLCDFYRMPRRVFNARMKAQSSISPGGSSGGSSGSDMPGTSESATPESSGGGSSGSARDTITKTLQLRIVRPYNSAEVEKIVADEKNNREKIALEKNKDKVREACSKHLKVASYCTTQVERNACPFCKARKLDDKFYQKLRGQFPDAVFWQEIGEIFRQLQKQAAEIYNQSLIELYYEIFIKGKGITNASRVEHYLSDVCYTRAAELFKNAAIASGLRSKVRSNFRLKELKNMKSGLPTTKSDNFPIPLVKQKGGQYTGFEISSHNSDFIIKIPFGRWQVKEEIDKYRPWEKFDFEQVRKSPKPISLLLSTQRRKKNKGWSKDEGTEAEIRKVMNGDYQTSYVEVKRGSKTGEKSAWMLNLSIDVPKIDKGVDPSIIGGIDVGVKSPLVCAIDNALSRYSISDNDLFRFNKKMFARRRILLKKNRHKRAGHGAKNKLKPISILTGKSERFRKKLIERWACEIADFFIKNKVGTVQMENLESMKRKEDSYFNIRLRGFWPYAEMQNKIEFKLKQYGIEIRKVAPNNTSKTCSKCGHLNNYFNFEYRKKNKFPHFKCEKCNFKENADYNAALNISNPRLKSTKEEP

SEQ ID NO: 2672 - protein, 726 aa, synthetic construct
SEVEFSHEYWMRHALTLAKRARDEREVPVGAVLVLNNRVIGEGWNRTTGLHDPTAHAEIMALRQGGLVMRNYRLTDATLYVTFEPCVMCAGAMIHSRIGRVVFGVRNSKRGAAGSLMNVLNYPGMNHRVEITEGILVDECAALLCDFYRMPRQVLNAQKKAQSSISPGGSSGGSSGSETPGASESATPESSGGSSGGSAKNTITKTLKLRIVRPYNSAEVEKIVADEKNSREKVALEKNKDKVKEACSEHLRVAAYCTTQVERNACLFCKARKLDDKFYQKLRGQFPDAVFWQEIGEIFRQLQKQAAEIYNQSLIELYYEIFIKGKGFANASSVEHYLSDVCYARAAELFKNAAIASGLRGKVKSNFRLKELKNMRSGLPTTKSDNFPIPLVKQKGGQYTGFEISSHNDDFIIKIPFGRWQVKKEIDKYRPWEKFDFEQVRKSPKPISLLLSTQRRKRNKGWSKDEGTEAEIRKVMNGDYQTSYIEVKRGSKTGEKSAWMLNLSIDVPKIDKGVDPCIIGGIDVGVKSPLVCAINNAFSRYSISDNDLFHFNKKMFARRRILLKENRHKRAGHGAKNKLKPITILTGKSRRFRKKLIERWACEIADFFIKNKVGTVQMESLESMKRKEDSYFNIRLRGFWPYAEMQNKIEFKLKQYGIKIRKVAPNNTSKTCSKCGHLNNYFSFEYRKKNKFPHFKCEKCNFKENADYNAALNISNPKLMSTKEEP

SEQ ID NO: 2673 - protein, 726 aa, synthetic construct
SEVEFSHEYWMRHALTLAKRARDGREVPVGAVLVLNNRVIGEGWNRAIGLHDPTAHAEIMALRQGGLVMQNYRLIDATLYVTFEPCAMCAGAMVHSRIGRVVFGVRNSKRGAAGSLMNVLTYPGMDHRVEITGGILADECAALLCDFYRMPRRVFNAQKKAQSSINSGGSSGGSSGSVTPGTSESATPESSGGSFGGTAKNTITKTLQLRIVRPYNSAEVEKIVADEKNSREKIALEKNKDKVKEACGKHLKAASYCTTQVERNACLFCKARKLDDEFYQKLRGQFPDAVFWQELGEIFRQLQKQAAEIYNQSLIELYYEIFIKGRGFANAGSVEHYLSDVCYTRAAELFKNAAIASGLRGKVKSNFRLKELKNMKSGLPTTKSDNFPIPLVKQKGGQYTGFEISSHNDDFIIKIPFGRWQVKKEIDKYRPWEKFDFEQVRKSPKPISLLLSTQRRKRNKGWSKDEGTEAEIRKVMNGDYQTSYIEVKRGSKTGEKSAWMLNLSIDVPKIDKGVDPSIIGGIDVGVKSPLVCAINNALSRYSISDNDLFHFNKKMFARRRILLKKNRHKRAGHGARNKLKPITVLTEKSERFRKKLIERWACEIANFFIKNKVGTVQMENLESMKRREDSYFNIRLRGFWPYAEMQSKIEFKLKQYGIEIRRVAPNNTSRTCSKCGHLNSYFNFEYRKKNKFPHFKCEKCNFREDADYNAALNISNPKLKSTKEEP

SEQ ID NO: 2674 - protein, 726 aa, synthetic construct; identical to SEQ ID NO: 684

SEQ ID NO: 2675 - protein, 726 aa, synthetic construct
SEVEFSHEYWMRHALTLAKRARDEREVPVGAVLVLNNRVIGEGWNRAIGLHDPTAHAEIMALRQGGLVMQNYRLIDATLYVTFEPCVMCAGAMIHSRIGRVVFGVRNSKHGAAGSLMNVLNYPGMNHRVEITEGILADECAALLCDFYRMPRQVFNARKKAQSSINPGGPSGGSSGSETPDTSESATPESSGGSSGSSAKNTITKTLKLRIVRPYNSAEVEKIVADEKNNREKIALEKNKDKVKEACSKHLKVAAYCTTQVERNACLFCKARKLDDKFYQKLRGQFPDAVFWQELGEILRQLQKQAAEIYNQSLIELYYEIFIKGRGFANASSVEHYLSDVCYTRAAELFKNAAIASGLRGKVKSNFRLKELKNMKSGLPTTKSDNFPIPLVRQKGGQYTGFEISSHNDDFIIKIPFGRWQVKEEIDKYRPWEKFDFEQVRKNPKPISLLLSTQRRKRNKGWSKDEGTEAEIRKVMNGDYQTSYIEVKRGSKIGEKSAWMLNLSIDVPKIDKGVDPSIIGGIDVGVKSPLVCAISNAFSRYSISDNDLYHFNKKMFARRRILLKKNRHKRAGHGAKNKLKPISILTGKSERFRKKLIERWACEIADFFIKNKVGTVQMENLESMKRKEDSYFNIRLRGFWPYAEMQNKIEFKLKQYGIKIRKVAPNNTSKTCSKCGHLNNYFSFEYRKKNKFPHFKCEKCNFKENADYNAALNISNPKLMGTKEEP

SEQ ID NO: 2676 - protein, 726 aa, synthetic construct
SEDEFSHEYWMRHALTLAKRARDEREVPVGAVLVLNNRVIGEGWNRAIGLHDPTAHAEIMALRQGGLVMQNYRLIDATLYVTFEPCVMCAGAMIHSRIGRVVFGVRNNKHGAAGSLVNVLNYPGMNHRVEITEGILADECAALLCDFYRMPRQVFNARKKAQSSINPGGSSGGSSGSETPGTSESATPESSGGSSGSSAKNTITKTLKLRIVRPYNSAEVEKIVADEKNNREKIALEKNKDKVKEACSKHLKVAAYCTTQVGRNACLFCKARRLDDKFYQKLRGQFPDAVFWQEIGEIFRQLQKQAAEVYNQSLVELYYEILIKGKGIANASSVEHYLSDVCYTRAAELFKNAAIASGLRNKIKSNFRLKELRNMKSGLPTTKSDNFPIPLVRQKGGQYTGFEISNHNSDFIIKIPFGRWQVKKEINKHRPWEKFDFEQVRRSPKPISLLLSTQRRKRNKGWSKDEGTEAEIRKVMSGDYQTSYIEVKRGSKIGEKSAWMLNLSIDVPKIDKGVDPSIIGGIDVGVKSPLVCAINNSFSRYSICDNDLFRFNKKMFARRRILLKKNRHNRAGHGAKNKLKPITILTEKSGRFRKKLIERWACEIADFFVKNKVGTVQMENLESMKRREDSYFNIRLRGFWPYAEMQNKVEFKLKQYGIKVRKVAPNNTSKTCSKCGHLNNYFSFEYRKKNKFPHFKCEKCNFKENADYNAALNISNPKLKSTKEEP

SEQ ID NO: 2677 - protein, 726 aa, synthetic construct
SEVEFSHEYWMRHALTLAKRARDEREVPVGAILVLNNRVIGEGWNRAIGQHDPTAHAEIMALRQGGLVMQNYRLIDATLYVTFEPCVMCAGAMIHSRIGRVVFGVRNSKHGAAGSLVNVLNYPGMNHRVETTEGILAEECAALLCDFYRMPRQVFNAQKKAQSTINSGSSSGGSSGSETPGTSESPTPESSGGIPGGSAKNTITKTLKLRIVRPYNSAEVEKIVADEKNNREMIALEKNKGKVKEACSKHLKVAAYCTTQVERNACLFCKARKLDDKFYRKLRGQFPDAVFWQEIGEIFRQLQRQAAEIYNQSLIELYYEIFIKGKGFANASSVEHYLSDVCYTRAAELFKNAAIASGLRGKVKGNFRLKELKNMKSGLPTTKSDNFPIPLVKQKGGQYTGFEISSHNDDFIIKIPFGRWQAKKEIDKYRPWEKFDFEQVRRSPKPISLLLSTQRRKRNKGWSKDEGTEAEIRKVMNGDYQTSYIEVKRGSKIGEKSAWMLNLSIDVPKIDKGVDPSIIGGIDVGVKSPLVCAINNAFSRYSISDNDLFHFNKKMFARRRILLKKNRHKRAGHGAKNKLKPISILTEKSKRFRKKLIERWACEIADFFIKNKVGTVQMENLESMKRKEDSYFNIRLRGFWPYAEMQNKIELKLKQYGIEIRRVAPNNTSRTCSKCGHLNNYFNFEYRKKSKFPLFKCEKCNFREDADYNAALNISNPKLKSTKEEP

SEQ ID NO: 2678 - protein, 726 aa, synthetic construct
SEVEFSHEYWMRHALTLAKRARDEREVPVGAILVLNNRVIGEGWNRAIGLHDPTAHAEIMALRQGGLVMQNYRLIDATLYVTFEPCVMCAGAMIHSRIGRVVFGVRNSKHGAAGSLVNVLNYPGMNHRVEITEGILADECAALLCDFYRMPRQVFNARKKAQSSINPGGSSGGSSGSETPGTSESPTPESSGGSSGGSAKNTITKTLKLRIVRPYNSAEVEKIVAEEKNNREKIALEKNKDKVKEACSKHLKVAAYCTTQVERNACLFCKARKLDDKFYQKLRGQFPDAVFWQEIGEIFRQLQKQAAEIYNQSLIELYYEIFIKGKGFANASSVEHYLSDVCYTRAAELFKNAAIASGLRGKVKSNFRLKELKNMKSGLPTTKSDNFPIPLVKQKGGQYTGFEISSHNDDFIIKIPFGRWQVKKEINKYRPWEKFDFEQVRKSPKPISLLLSTQRRKRNKGWSKDEGTEAEIRKVMNGDYQTSYIEVKRGSKIGEKSAWMLNLSIDVPKIDKGVDPSIIGGIDVGVKSPLVCAISNAFSRYSISDNDLFHFNKKMFARRRILLKKSKHKRAGHGAKNKLKPITILTEKSRRFRKKLIERWACEIADFFIRNKVGTVQMENLESMKRKEDSYFNVRLRGLWPYAEMQNKIELKLKQYGIEIRKVAPNNTSKTCSMCGHLNNYFNFEYRKKNKFPHFKCEKCNFKEDADYNAALNISNPMLKSTKEEP

SEQ ID NO: 2679 - protein, 726 aa, synthetic construct
SEVEFSHEYWMRHALTLAKRARDEREVPVGAVLVLNNRVIGEGWNRAIGLYDPTAHAEIMALRQGGLVMQNYRLIDATLYVTFEPCVMCAGAMIHSRVGRVVFGVRNSKHGAAGSLMNVLNYPGMNHRVEITEGILADECAALLCDFYRMPRRVFNARRKAQSSIDPGGPSGGSSGSETPGTSESATPESSGGSSGGSAKNTITKTLKLRIVRPYNSTEVEKIVADEKNNREKIALEKNKDKVKEACSKHLKVAAYCTTQVERNACLFCKARKLDDKFYQKLRGQFPDAVFWQEIGEIFRQLQKQAAEIYNQSLIELYYEILIKGKGIANASSVEHYLSDVCYTRAAELFKNAAIASGLRNKIKSNFRLKELRNMKSGLPTTKSDNFPIPLVRQKGGQYTGFEISNHDGDFIIKIPFGRWQVKKEINKHRPWEKFDFGQVRKSPKPISLLLSTQRRKRNKGWSKDEGTEAEVRKVMNGDYQTSYIEVKRGSKIGEKSAWMLNLSIDVPKIDKGVDPSIIGGIDVGVKSPLVCAINNALSRYSISDNDLFHFNKKMFARRRILLRKNRHKRAGHGAKNKLKPITIMTEKSKRFRKKLIERWACEIADFFTKNKVGTVQMENLESMKRKEDSYFNIRLRGFWPYAEMQNKIEFKLKQYGIVVRKVAPNNTSKTCSKCGHLNNYFNFEYRKKNKFPHFKCEKCNFKEDADYNAALNISNPKLKSTKEEP

SEQ ID NO: 2680 - protein, 726 aa, synthetic construct
SEVEFSHEYWMRHALTLAKRARDEREVPVGAVLVLNNRVIGVGWNRAIGLHDPTAHAEIMALRQGGLVMQNYRLIDATLYVTFEPCVMCAGAMIHSRIGRVVFGVRNSKRGAAGSLMNVLNYPGMNHRVEITEGVLADECAALLCDFYRMPRQVLNAQKKAQSSINSGGSSGGGSGGETPGTSESATQESSGGSSGGSAKNTITKTLKLRIVRPYNSAEVEKIVADEKNNREKIALEKNKDKVKEACSKHLKVAAYCTTQVERNACLFCKARKLDDKFYQKLRGQFPDAVFWQEISEIFRQLQKQAAVVYNQGLIELYYEIFIKGKGIANASRVEHYLSNVCYTRAAELFKNAAIASGLRSKIKSNFRLKELKNMKSGLPTTKSDNFPIPMVKQKGGQCTGFEISNHNGDFIIKIPFGRWQVKKGIDKYRPWEKFDFEQVRKSPKPISLLLSTQRRRRNKGWSKDEGTEAEIKKVMNGDYQASYIEVKRGSKIGEKSAWMLNLSIDVPKIDKGVDPSIIGGIDVGVKSPLVCAINNAFSRYSISDNDLFHFNKKVFARRRILLKKNRHKRAGHGAKNKLKPITILTGKSKRFRKKLIERWACEIADFFIKNKVGTVQMENLESMKRKEDSYFNIRLRGFWPYAEMQNKIEFKLEQYGIEIRKVAPNNTSRTCSKCGHLNNYFNFEYRKKNKFPHFKCEKCNFKENADYNAALNISNPKLKSTKEEP

SEQ ID NO: 2681 - protein, 726 aa, synthetic construct; identical to SEQ ID NO: 684

SEQ ID NO: 2682 - protein, 726 aa, synthetic construct
SEVEFSHEYWMRHALTLAKRARDEREVPVGAVLVLNNRVIGEGWNRAIGLHDPTAHAEIMALRQGGLVMQNYRLVDATLYVTFEPCVLCAGAMVHSRIGRVVFGVRNSKRGAAGSLMNVLNYPGMNHRVEITEGILADECAALLCDFYRMPRQVFNARKKAQSSISPGGSSGGCSGSEMPGASESVTPKSSGGSSAGSTKNTITKTLKLRIVRPYNSAEVEKIVADEKNSREKIALERNKDKVKEACSEHLKVAAYCTTQVERNACLFCKARKLDDRFYQKLRGQFPDAVFWQETGEIFRQLQRQAAEIYNQSLIELYYEIFIKGKGFANASSVEHYLSDVCYTRAAELFKNAAIASGLRGKVKSNFRLKELKNMRSGLPTTKSDNFPIPLVKQKGGQYTGFEISSHNDDFIIKIPFGRWQVKKEIDKYRPWERFDFEQVRKSPKPISLLLSTQRRKRNKGWSKDEGTEAEIRKVMNGDYQTSYIEVKRGSKIGEKSAWMLNLSIGVPKIDKGVDPSIIGGIDVGVKSPLVCAINNAFSRYSISDNDLFHFNKKMFARRRILLKKNRHKRAGHGAKNKLKPITVLTEKSERFRKKLIEKWACEIADFFIKNKVGTVQMENLESMKRKEDSYFNIRLRGFWPYAEMQNKIEFKLKQYGIETRKVAPNNTSKTCSKCGHLNNYFNFEYRKKNKFPHFKCEKCNFKEDADYNAALNISNPKLKSTKEEP

SEQ ID NO: 2683 - protein, 726 aa, synthetic construct
GEVEFSHEYWMRHALTLAKRARDEREVPVGAVLVLNNRVIGEGWNRAIGLHDPTAHAEIMALRQGGLVMQNHRLADATLYVTFEPCVLCAGAMVHSRIGRVVFGVRNSKRGAAGSLMNVLNYPGMNHRVEITEGILADECAALLCDFYRMPRQVFNAQKKAQSSISSGGSSGGSSGSETPGAGESVTPKSSVGSSAGSTKNTITKTLKLRIVRPYNSAEVEKIVADEKNNREKFALEKNKDKVKEACSKHLKVAAYCTTQVERNACLFCKARKLDDKFYQKLRGQFPDAVFWQEVGEIFRQLQKQAAEIYNRSLIELYYEIFIKGKGFANASSVEHYLSDVCYTRAAELFKNAAIASGLRGKVKSNFRLKELKNMKSGLPTTKSDNFPIPLVRQKGGQYTGFEISNHDGDFIIKIPFGRWQVKKEINKHRPWEKFDFEQVRKSPKPISLLLSTQRRKRNKGWGKDEGTEAEIRKVMNGDYQTSYIEVKRGNKTGEKSAWMLNLSIDVPKIDKGVDPSIIGGIDVGVKSPLVCAVNNSFSRYSICDNDLFRFNKKMFARRRILLKKNRHRRAGHGAKNKLKPITILTEKSVRFRKKLIERWACEIADFFIKNKVGTVQMENLESMKRKEDSYFNIRLRGFWPYAEMQNKIEFKLKQYGIEIRKVAPNNTSKTCSKCGHLNNYFNFEYRKKNKFPHFKCEKCNFKENADYNAALNISNPKLKSTKGEP

SEQ ID NO: 2684 - protein, 726 aa, synthetic construct
SEVEFSHEYWMRHALTLAKRARDEREVPVGAVLVLNNRVIGEGWNRAIGLHDPTAHAEVMALRQGGLVMQNYRLTDATLYVTFEPCVMCAGAMIHSRIGRVVFGVRNSKRGAAGSLMNVLNYPGMNHRVEITEGILVDECAALLCDFYCMPRQVLNAQKKAQSSISPGGSSGGSSGSETPGTSESPTPESSGGSPGGSAKSTITKTLKLRIVRPYNSAEVEKIVADEKNNREKIALEKNKDKVKEACSKHLKVAAYCTTQVERNACLFCKARKLDDKFYQKLRGQFPDAVFWQEIGEIFRQLQKQAAEIYNQSLIELYYEIFVKGKGFANASSVEHYLSDVCYTRAAELFKNAAIASGLRGKVKSNFRLKELKNMKSGLPTTKSDNFPIPLVRQKGGQYTGFEISNHDGDFIIKIPFGRWQVKKEINKHRPWEKFDFEQVRKSPKPISLLLSTQRRKRNKGWSKDEGTEAEIRKVMNGDYQTSYIEVKRGSKIGEKSAWMLNLSIDVPKIDKGVDPSIIGGIDVGVKSPLVCAINNAFSRYSISDNDLFHFNKKVFARRRILLKKNRHRRAGHGAKNKLKPITILTEKSKRFRKKLIERWACEIADFFIKNKVGTVQMENLESMKRKEDSYFNVRLRGFWPYAEMQNKIEFKLKQYGIKIRKVAPNNTSRTCSECGHLNNYFSFEYRKKNKFPHFKCEKCNFKEDADYNAALNISNPKLKGTKEEL

SEQ ID NO: 2685 - protein, 726 aa, synthetic construct
SEDEFSHEHWMRHALTLAKRARDEHEVPVGAVLVLDNRVIGEGWNRAIGLHDPTAHAEIMALRQGGLVMQNYRLVDATLYVTFEPCVLCAGAMVHSRIGRVVFGVRNSKRGAAGSLLNVLNYPGMNHRVEITEGILADECAALLCDFYRMPRQVFSAQKKAQSSINSGGSSGGSSGSKTPGTSESATPESSGGSSSGSTKNTITKTLKLRIVRPYNSTEVEKIVADEKNNREKIALEKNKDKVKEACSRHLKVAAYCTTQVERNACLFCKARKLDDKFYQKLRGQFPDAVFWQEIGEIFRQLQKQAAEVYNQSLVELYYEIFIKGKGFANASSVEHYLSDVCYARAAELFKNAAIASGLRGKVKSNFRLKELKNMKSGLPTTKSDNFPIPLVKQKGGQYTGFEISNHSDDFIIKIPFGRWQVKEEIDKYRPWEKFDFEQVRKSPKPISLLLSTQRRKRNKGWSKDEGTEAEIRRVMNGDYQTSYIEVKRGSKIGEKSAWMLNLSIDVPKIDKGVDPSIIGGIDVGVKSPLVCAINNAFSRYSISDNDLFHFNKKMFARRRILLKKNRHKRAGHGAKNKLKPITILTEKSKRFRKKLIERWACEIADFFIKNKVGTVQMENLESMKRKEDSYFNIRLRGFWPYAEMQDKIEFKLKQYGIGIRKVAPNNTSKTCSRCGHLNNYFNFEYRKKNKFPHFKCEKCNFKENADYNAALNISNPKLKSTKEEP

SEQ ID NO: 2686 - protein, 726 aa, synthetic construct
SEVEFSHEYWMRHALALAMRARDEREVPVGAVLVLNNRVIGGGWNRTIGLHDPTAHAEIMALRQGGLVMQNCRLVDATLYVTFEPCVMCAGAMIHSRIGRVVFGVRNSKRGAAGSLVNVLNYPGMGHRVEIMEGILVDECAALLCDFYRMPRQVFNAQKRAQSTINSGGSSGGSSGSETPGTSESPTPESSGGSPGGSAKNTITKTLKLRIVRPYNSAEVEKIVADEKNNREKIALEKNKDKVKEACRKHLKVATYCTTQVERNACLFCRARKLDDKFYQKLRGQFPDAVFWQEIGEIFRQLQRQAAEIYNQSLIELYYEIFIKGKGFANASSVEHYLSDVCYTRAAELFKNAAIASGLRGKVKSNFRLKELKNMKSGLPTTKSDNFPIPLVKQKGGQYTGFEISSHNDDFIIKIPFGRWQVKKEIDKYRPWEKFDFEQVRKSPKPISLLLSTQRRKRNKGWSKDEGTEAEIRKVMNGDYQTSYIEVKRGSKIGEKSAWMLYLSIDVPKIDKGVDPSIIGGIDVGVKSPLVCAIYNAFSRYSIGDNDLFHYNKKMFARRRILLKKNRHKRAGHGAKNKLKPISILTEKSKRFRKKLIERWACEIADFFIKNKVGTVQIENLESMKRKEDSYFNIRLRGFWPYAEMQNKIEFKLKQYGIEIRKVAPNNTSKTCSKCGHLNSYFNFEYRKKNKFPHFMCEKCNFKEDADYNAALNISNPKLKSTKEEP

SEQ ID NO: 2687 - protein, 726 aa, synthetic construct
SEVEFSHEYWMRHALTLARRARDEREVPVGAILVLNNRVIGEGWNRAIGLHDPTAHAEIMALRQGGLVMQNYRLIDATLYVTFEPCAMCAGAMIHGRIGRVVFGVRNNKHGAAGSLMNVLNYPGMDHRVEITEGILADECAALLCDFYRMPRQVFNARKKAQSSINPGGSPGGSSGSETPGTSESATLESSGGGFGGSTKNTITKTLKLRIVRPYNSAEVEKIVADEKNSREKIALEKNKGKVKEACSKHLEVAAYCTTQVERNACLFCKARKLDDKFYQKLRGQFPDAVFWQELGEIFRQLQKQAAEIYNQSLIELYYEIFIKGKGFANASSVEHYLSDVCYTRAAELFKNAAIASGLRGKVKSNFRLKELKNMKSGLPTTKSDNFPIPLVKQKGGQYTGFEVSSHNDDFIIKIPFGRWQVKKEIDKYRPWEKFDFEQVRKSPRPISLLLSTQRRKRNKGWSKDEGTEAEIRKVMNGDYQTSYIEVKRGSKTGEKSAWMLNLSIDVPKIDKGVDPSIIGGIDVGVKSPLVCAINNAFSRYSISDNDLFHFNKKMFARRRILLKKTRHKRAGHGAKNKLKPISILTEKSERFRKKLIERWACEIADFFVKNKVGTVQMENLESMKRREDSYFNIRLRGFWPYAKMQNKIEFKLKQYGIEIRKVAPNNTSKTCSKCGHLNNYFNFEYRKKNKFPHFKCEKCNFKENADYNAALNISSPKLKSTKEEP

SEQ ID NO: 2688 - protein, 726 aa, synthetic construct
SEGEFSHEYWMRHALALAKRARDEREVPVGAVLVLNNRVIGEGWNRAIGLHDPTAHAEIMALRQGGLVMQNHRLVNATLYVTFEPCVMCAGAMIHSRIGRVAFGVRNSKRGAAGSLMNVLNYPGMNHRVEITEGILAAECAALLCDFYRMPRQVFNAQKKAQSNINSDGSSGGSNGSETPGTSGSPTPESSGGSSGGSAKNTITKTLKLRIVRPYNSAEVEKIVADEKNNREKIALEKNKDKVKEACSKHLKVAAYCTTQVERNACLFCKARKLDDKFYQKLRGQFPDAVFWQEIGEIFRQLQKQAAEVYNQSLVELYYEILIKGKGIANASSMEHYLSDVCYTRAAELFKNAAIASGLRNKIKSNFRLKELRNMKSGLPTTKSDNFPIPLVRQKGGQYTGFEISNHDGDFIIKIPFGRWQVKKEINKHRPWEKFDFEQVRKSPKPISLLLSTQRRKRNKGWSKDEGTEAEIRKVMNGDYQTSYIEVKRGSKIGEKSAWMLNLSIDVPKIDKGVDPSIIGGIDVGVKSPLVCAINNASSRYSISDNDLFHFNKKMFARRRILLKKNRHKRAGHGAKNKLKPISILTEKSKRFRKKLIERWACEIADFFIKNKVGTVQMENLESMKRKEDSYFNIRLRGFWPYAEMQNKIEFKLKQYGIEIRKVAPNNTSKTCSKCGHLNNYFNFEYRKKNKFPHFKCEKCNFRENADYNAALNISNPKLRSTKEEP

SEQ ID NO: 2689 - protein, 726 aa, synthetic construct
SEVEFSHEYWMRHALTLAKRARDEREVPVGAILVLNNRVIGEGWNRAIGLHDPTAHAEIMALRQGGLVMQNYRLIDATLYVTFEPCVMCAGAMIHSRIGRVVFGVRNNKHGAAGSLVNVLNYPGMNHRVEITEGILADECAALLCDFYRMPRQVFNARKKAQSSTNPGGSSGGSGGSVTPGTSESATPESSGGSSGGSAKNTITKTLKLRIVRPYNSAEVEKIVADEKNNREKIALEKNKDKVKEACSKHLKVASYCTTQVERNACPFCKARKLDDKFYQKLRGQFSDAVFWQELGEIFRQLQKQAAEIYNQSLIELYYEIFIKGRGFANASSVEHYLSDVCYTRAAELFKNAAIASGLRGKVKSNFRLKELKNMKSGLPTTKSDNFPIPLVKQKGGQYTGFEISSHHDDFIIKIPFGRWQVKKEIDKYRPWEKFDFEQVRKSPKPISLLLSTQRRKRNKGWSKDEGTEAEIRKVMNGDYQTSYIEVKRGSKIGEKSAWMLNLSIDVPKIDKGVDPSIIGGIDVGVKSPLVCAINNAFSRYSISDNELFHFNKKMFARRRILLKKSRHKRAGHGAKNKLKPISILTGKSERFRKKLIERWACEIADFFTKNKVGTVQMENLESMKRREDSYFNIRLRGFWPYAEMQNKIEFKLKQYGIEIRKVAPNNTSKTCSKCGHLNNYFNFEYRKKNKFPHFKCEKCNFKENADYNAALNISNPKLKGTKEEP

SEQ ID NO: 2690 - protein, 726 aa, synthetic construct
SEVEFSHEYWMRHALTLARRARDEREVPVGAILVLNNRVIGEGWNRAIGLHDPTAHAEIMALRQGGLVLQNYRLIDATLYVTFEPCVMCAGAMIHSRIGRVVFGVRNNKHGAAGSLVNVLNYPGMNHRVEITEGILADECAALLCDFYRMPRLVFNARKKTQSSINPGGSSGDSSGSETPGTSESATPESSGGSSGSSAKNTITKTLKLRIVRPYNSAEVEKIVADEKNNREKIALEKNKDKVKEACSKHLKVAAYCTTQVERNACLFCKARRLDDKFYQKLRGQFPDAVFWQEIGEIFRQLQKQAAEVYNQSLVELYYEILIKGKGIANASSVEHYLSDVCYTRAAELFKNAAIASGLRNKIKSNFRLKELRNMKSGLPTTKSDNFPIPLVRQKGGQYTGFEISNHDGDFIIKIPFGRWQVKKEIDKYRPWEKFDFEQVRKSPKPISLLLSTQRRKRNKGWSKDEGTEAEIRKVMNGDYQTSYIEVKRGSKIGEKSAWMLSLSIDVPKIDKGVDPSIIGGIDVGVKSPLVCAINNALSRYSISDNDLFRFNKKMFARRRILLKRNRHKRAGHGTKNKLKPITILTEKSGRFRKKLIERWACEIADFFIKNKVGTVQLENLESMKRREDSYFNIRLRGFWPYAEMQNKIEFKLRQYGIEIRKVAPNNTSKTCSKCGHLNNYFDFEYRKKNKFPHFKCEKCNFKENADYNAALNISNPKLRSTKEEP

SEQ ID NO: 2691 - protein, 726 aa, synthetic construct
SEVEFGHEYWMRHALTLAKCARDEREVPVGAILVLNNRVIGEGWNRAIGLHDPTAHAEIMALRQGGLVMQNYRLIDATLYVTFEPCVMCAGAMIHSRIGRVVFGVRNNKHGAAGSLVNVLNYPGMNHRVEITEGILANECAALLCDFYRMPRQVFNARKKAQSSINPGGSSGGSSGSETPGTSESATPESSGGSSGGSAKNTITKTLKLRIVRPYNSAEVEKIVADEKNNREKIALEKNKDKVKEACSKHLKVAAYCTTQVERNACLFCKARRLDDKFYQKLRGQFPDAVFWQEIGEIFRQLQKQAAEIYNQSLVELYYEILIKGKGIANASSVEHYLSDVCYTRAAELFKNAAIASGLRNKIKSNFRLKELRNMKSGLPTTKSDNFPIPLVRQKGGRYTGFEISNHNGDFIIKIPFGRWQVKREINKHRPWEKFDFEQVRKSPKPISLLLSTQRRKRNKGWSKDEGTEAEIRKVMNGDYQTSYIEVKRGSKIGEKSAWMLNLSIDVPKIDKGVDPSIIGGIDVGVKSPLVCAISNAFGRYSISDNDLFHFNKKMFARRRILLKKNRHKRAGHGAKNKLKPITILTEKSKRFRKKLIERWACEIADFFIKNKVGTVQMENLESMKRKEDSYFNIRLRGFWPYAEMQDKIEFKLKQYGIEIRKVAPNNTSKTCSKCGHLNNYFNFEYRKKNKFPHFKCEKCNFKENADYNAALNISNPKLKSTKGEP

SEQ ID NO: 2692 - protein, 726 aa, synthetic construct
SEVEFSHEYWMRHALTLAKRARDEREVPVGAVLVLNNRVIGGGWNRAIGLHDPTAHAEIMALRQGGLVMQNCRLVDATLYVTFEPCVMCAGAMIHSRIGRVVFGVRNSKRGAAGSLMNVLNYPGMNHRVEITGGVLADECAALLCDFYRMPRQVFNAQKKAQSSISSGGSSGGSSGSETPGASGSVTPKSSGGSSGGSAKNTITKTLKLRIVRPYNSAEVEKIVADEKNNREKIALEKNKNKVKEACSKHLKVAAYCTTQVERNACQFCKARKLDDKFYQKLRGQFPDAVSWQEIGEIFRQLQKQAAEIYNQSLIELYYEIFIKGKGFANASSVEHYLSDVCYTRAAELFKNAAIASGLRGKVKSNFRLKELKSMKSGLPTTKSDNFPIPLVKQKGGQYTGFEINSHNDDFIIKIPFGRWQVKREIDRYRPWEKFDFEQVRKSPKPISLLLSTQRRKRNKGWSKDEGTEAEIRKVMNGDYQTSYIEVKRGSKIGEKSAWMLSLSIDVPKIDKGVDPSTIGGIDVGVKSPLVCAINNAFCRYSISDNDLFHFNKKMFARRRILLKKNRHKRAGHGAKNKLKPISILTEKSKRFRKKLIERWACEIADFFIKNKVGTVQMENLESMKRKEDSYFNIRLRGLWPYAEMQNKIEFKLKQYGIKIRKVAPNNTSRTCSKCGHLNNYFNFEYRKKNKFPHFKCEKCSFKENADYNAALNISNPKLKSTKEEP

SEQ ID NO: 2693 - protein, 726 aa, synthetic construct
SEVEFSHEYWMRHALTLAKRARDEREVPVGAVLVLNNRVIGEGWNRAIGLHDPTAHAEIMALRQGGLVMQNCRLSDATLYVTFEPCAMCAGAMIHSRIGRVVFGVRNSKRGAAGSLMNVLNYPGMNHCVEITEGILVDECAALLCDFYRMPRQVLSAQKKAQSTINSGGSSGGSSGSETPGTSESPTPESSGGSPGGSAKNTITKTLKLRIVRPYNSAEVEKIVADEKNNREKIALERNKDKVKEACSKHLGVAAYCTTQVERNACLFCKARKLDDKFYQKLRGQFPDAVFWQELGEIFRQLQKQAAEIYNQSLIELYYEIFIKGKGFANASSVEHYLSDVCYTRAAELFRNAAIASGLRGKVKSNFRLKELKNMKSGLPTTKSDNFPIPLVKQKGGQYTGFEISSHNSDFIIKIPFGRWQVKEEIDKYRPWEKFDFEQVRKSPKPISLLLSTQRRKRNKGWSEDEGTEAEIRKVMNGDYQTSYIEVKRGSKIGEKSAWMLNLSIDVPKIDKGVDPSIVGGIDVGVKSPLVCAIDNALSRYSISDNDLFHFNKKMFARRRILLKKNRHRRAGHGVKNKLKPVSILTEKSKRFRKKLIERWACEIADFFIKNKVGTVQMENLESMKRKEDSYFNIRLRGFWPYAEMQNKIEFKLKQYGIEIRKVAPNNTSKTCSKCGHLNNYFTFEYRKKNKFPHFKCEKCNFKEDADYNAALNISNPKLKSTKEEP

SEQ ID NO: 2694 - protein, 726 aa, synthetic construct
SEVEFSHEYWMRHALTLAKRARDEREVPVGAVLVLNNRVIGEGWNRAIGLHDPTAHAEIMALRQGGLVMQNYRLIDATLYVTFEPCVMCAGAMIHSRIGRVVFGVRNNKHGAAGSLVNVLNHPGMNHRVKITEGILADECAALLCDFYRMPRRVFNAQKKVQSSINSGGSSGGGSGSETPSTSENTTPESSGGSSGGPAKNTITKTLKLRIVRPYNSAEVEKIVADEKNNREKTALEKNKDKVKEACSKHLKVAAYCTTQVERNACLFCKARKLDDKFYQKLRGQFPDAVFWQEVGEIFRQLQKQAAEIYNQSLIELYYEIFIKGKGFANASSVEHYLSDVCYTRAAELFKNAAIASGLRGKVKSNFRLKELKSMKSGLPTTKSDNFPIPLVKQKGGQYTGFEISSHNDDFIIKIPFGRWQVRKEIDKYRPWEKYNFEQVRKSPKPISLLLSTQRRKRNKGWSKDEGTEAEIRKVMNGDYQTSYIEVKRGSKIGEKSAWMLNLSIDVPKIDKGVDPSIVGGIDVGVKSPLVCAIDNVLSRYSISDNDLFHFNKKMFARRRILLKKNRHRRAGHGAKNKLKPISILTEKSKRFRKKLIERWACEIADFFIKNKVGTVQMENLESMKRKEDSYFNIRLRGFWPYAEMQNRIEFKLKQHGIEIRKVAPNNTSKTCSKCGHLNNYFSFEYRKKNKFPHFKCEKCNFKENADYNAALNISNPKLKSTKEEP

SEQ ID NO: 2695 - protein, 726 aa, synthetic construct
SEVEFSHEYWMRHALTLAKRARDEREVPVGAVLVLNNRVIGEGWNRAIGLHDPTAHAEIMALRQGGLVMQNYRLTDATLYVTFEPCVMCAGAMIHSRIGRVVFGVRNSKRGAAGSLMDVLNYPGMNHRVEITEGILADECAALLCDFYRMPRQVFSAQKKAQSSIDSGGSSGGSSGSITPGTSESATPESSGGGSGGSAQNTITKTLKLRIVRPYNSAVVEKIVADEKNNREKIALERNKDKVKEACSKHLKVAAYCTTQVERNACLFCKARKLDDKFYQKLRGQFPDAVFWQEISEIFRQLQKQAAEIYNQSLIELYYEIFIKGKGIASASRVGHYLSDVCYTRAAELFKNAAIASGLRSKIKSNFRLKELKNMKSGLPTTKSDNFPIPLVKQKGGQYTGFEISSHNDDFIIKIPFGRWQVKKEIDKYRPWEKFDFEQVRRSPKPISLLLSTQRRKRNKGWSKDEGTEAEIRKVMNGDYQTSYIEVKRGSKIGEKSAWMLNLSIDVPKIDRGVDPSIIGGIDVGVKSPLVCAINNAFSRYSISDNDLFRFNKKVFARRRILLKKNRHKRAGHGTKNKLKPITILTEKSGRFRRKLIERWACEIADFFIKNKVGTVQMENLESMKRKEDSYFNIRLRGFWPYAEMQNKIEFKLKQYGIEIRKVAPNNTSKTCSKCGHLNNYFNFEYRKKNKFPHFKCEKCNFKENADYNAALNISNPKLKSTKEEP

SEQ ID NO: 2696 - protein, 726 aa, synthetic construct
SEVEFSHEYWMRHALTLAKRARDEREVPVGAILVLNNRVIGEGWNRAIGLHDPTAHAEIMALRQGGLVMQNYRLIDATLYVTFEPCVMCAGAMIHSRIGRVVFGVRNNKHGAAGSLVNVLNYPGMNHRVEITEGILADECAALLCDFYRMPRQVFNARKKAQSSINPGSPSGGSSGSETPDTSESATPESSGGSSGGSAKNTITKTLKLRIVRPYNSTEVEKIVADEKNNREKIALEKNKDKVKEACSKHLKVAPYCTTQVERNACLFCKARKLDDKFYQKLRGQFPNAVFWQELGEIFRQLQKQAAEIYNQSLIELYYEIFIKGKGFANASSVEHYLSDVCYTRAAELFKNAAIASGLRGKVKSNFRLKELKNMKSGLPTTKSDNFPIPLVKQKGGQYTGFEISSHNDDFIIKIPFGRWQAKKEINKHRPWEKFDFEQVRKSPKPISLLLSTQRRKRNKGWSKDEGTEAEIRKAMNGDYQTSYIEVKRGSKIGEKSAWMLSLSIDVPKIDKGVDPRIIGGIDVGVKSPLVCAINNVLSRYSISDNDLFHFNKKMFARRRILLKKNGHKRAGHGAKNKLKPITIMTEKSKRFRKKLIERWACEIADFFIKNKVGTVQMENLESMKRKEDSYFNIRLRGFWPYAEMQNKIEFKLRQYGIVVRKVAPNNTSKTCSQCGHLNNYFNFEYRKKNKFPYFKCEKCNFKENADYNAALNISNPQLKSTKGEP

SEQ ID NO: 2697 - protein, 726 aa, synthetic construct
SEVEFSHEYWMRHALTLAKRARDGREVPVGAVLVLNNRVIGEGWNRAIGLHDPTAHAEIMALRQGGLVMQNYRLIDATLYVTFEPCVMCAGAMVHSRIGRVVFGVRNSKRGAAGSLMNVLDYPGMGHRVEITEGILADECAALLCDFYCMPRQVFNAQKRAQSSINSGGSSGGSSGSETPGTSESATPESSGGGSSGSAKNTFTKTLQLRIVRPYNSAEVEKIVADEKDNREKIALEKNKDKVREACSRHLKVASYCTTQVERNACPFCKARKLDDKFYQKLRGQFSDAVFWQELGEILRQLQKQAAEIYNQSLVELYYEIFIKGRGFANASSVEHYLSDVCYTRAAELFKNAAIASGLRGKVKSNFRLKELKNMKSGLPTTKSDNFPIPLVKQKGGQYTGFEISSHNDDFIIKIPFGRWQVKKEIDKYRPWEKFDFEQVRKSPKPISLLLSTQRRKRNRGWSKDEGTEAEIRKVMNGDYQTSYIEVKRGSKTGEKSAWMLNLSIDVPKIDKGVDPSIIGGIDVGVKSPLVCAINNAFSRYSISDNDLFRFNKKMFARRRILLKKNRHKRAGHGAKNKLKPITILTEKSGRFRKKLIERWACEIADFFVKNKVGTVQMENLESMKGKEDSYFNIKLRGFWPYAEMQNKIEFKLKQYGIEIRKVAPNNTSKTCSKCGHLNNYFNFEYRKKNKFPHFKCEKCNFKENADYNAALNISNPKLKSTKEEP

SEQ ID NO: 2698 - protein, 726 aa, synthetic construct
SEVEFSHEYWMRHALTLAKRARDEREVPVGAVLVLNNRVIGEGWNRAIGLHDPTAHAEIMALRQGGLVMQNYRLIDATLYVTFEPCVMCAGAMVHSRIGRVVFGVRNSKRGAAGSLMNVLDYPGMGHRVEITEGILADECAALLCDFYCMPRQVFNAQKRAQSSINSGGSSGGSSGSETPGTSESATPESSGGGFGGSAKNTITKTLQLRIVRPYNSAEVEKIVADEKNNREKIALEKNKGKVKEACSKHLKVATYCTTQVERNACLFCKARKLDDKFYQKLRGQFPDAVFWQETGEIFRQLQRQAAEIYNQSLIELYYEIFIKGKGFANASSVEHYLSDVCYTRAAELFKNAAIASGLRGKVKSNFRLKELKNMKSGLPTTKSDNFPIPLVRQKGGQYTGFEISSHNDDFIIKIPFGRWQVKKEIDKYRPWEKFDFEQVRKNPKPISLLLSTQRRKRNKGWSKDEGTEAEIRKVMNGDYQTSYIEVKRGSRIGEKSAWMLNLSIDVPKIDKGVDPSIIGGIDVGVKSPLVCAINNAFSRYSISDNDLFRFNKKVFARRRILLKKNRHKRAGHGTKNKLKPITILTEKSGRFRKKLIERWACEIANFFIKNKVGTVQMENLESMKRKEDSYFNIRLRGFWPYAEMQNKIEFKLKQYGIKIRKVAPNNTSKTCSKCGHLNNYFSFEYRKKNKFPHFKCEKCNFKEDADYNAALNISNPNLKSTKEEP

SEQ ID NO: 2699 - protein, 727 aa, synthetic construct
SEVEFSHEYWMRRALTLAKRARDEREVPVGAVLVLNNRVIGVGWNRAVGLHDPTAHAEIMALRQGGLVMQNYRLIEATLYVTFEPCIMCAGAMIHSRIGRVVFGVRNSKRGAAGSLMNVLNYPGMNHRVEITEGILADECAALLCDYYRMPRQVFNARKKAQSSTNSGGSSDGGSGSETPGTSESATPESSGGSSGGSAKNTITKTLKLRIVRPYNSAEVEKIVADEKSNREKIALEKNKDKVKEACSEHLKVAAYCTTQVGRNACLFCKARRLDDKFYQKLRGQFPDAVFWQEIGEIFRQLQKQAAEVYNQSLVELYYEILIKGKGIANASSVEHYLSDVCYTRAAELFKNAAIASGLRNKIKSNFRLKELRNMKSGLPTTKSDNFPIPLVRQKGGQYTGFEISNHDGDFIIKIPFGRWQVKKEINKHRPWEKFDFEQVRRSPKPISLLLSTQRRKRNKGWSKDEGTEAEIRKVMNGDYQTSYIEVKRGSKIGEKSAWMLNLSIDVPKIDKGVDPSIIGGIDVGVKSPLVCAINNALSRYSISDNDLFHFNKKMFARRRILLRKNRHKRAGHGAKNKLKPITIMTEKSKRFRKKLIERWACEIADFFIKNKVGTVQMENLESMKRKEDSYFNIRLRGFWPYAEMQNRIELKLKQYGIEIRRVAPNNTSKTCSKCGHLNNYFNFEYRKKNKFPHFKCEKCNFKENADYNAALNISNPKLKSTKEEPQ

SEQ ID NO: 2700 - protein, 726 aa, synthetic construct
SEVEFSHEYWMRHALTLAKRARDEREVPVGAILVLNNRVIGEGWNRAIGLHDPTAHAEIMALRQGGLVMQNYRLIDATLYVTFEPCVMCAGAMIHSRIGRVVFGVRNSKHGAAGSLMNVLNYPGMNHRVEITEGILADECAALLCDFYRMPRQVFNARKKAQSSINPGGSSGGSSGSETPGTSESATPESSGGSSGSSAKNTITKTLKLRIVRPYNSAEVEKIVADEKNNREKIALEKNKDKVKEACSKHLKVAAYCTTQVERNACLFCKARRLDDKFYQKLRGQFPDAVFWQEIGEIFRQLQKQAAEIYNQCLIELYYEIFIKGKGFANASSVEHYLSDVCYTRAAELFKNAAIASGLRGKVKSNFRLKELKNMKSGLPTTKSDNFPIPLVRQKGGQYTGFEISNHNGDFIIKIPFGRWQVKKEISKHRPWEKFDFEQVRKSPKPISLLLSTQRRKRNKGWSKDEGTEAEIRKVMNGDYQTSYIEVKRGSKFGEKSAWMLNLSIDVPKIDKGVDPSIIGGIDVGVKSPLVCAINNAFSRYSISDNDLFRFNKKMFARRRILLGKNRHKRAGHGVKNKLKPITILTEKSERFRKKLIERWACEIADFFIKNKVGTVQMENLESMKRKEDSYFNIRLRGFWPYAEMQNKIEFKLKQYGIEIRKVAPNNTSRTCSKCGHLNNYFNFEYRKKNKFPHFKCEKCNFKENADYNAALNICNPKLKSTKEEP

SEQ ID NO: 2701 - protein, 726 aa, synthetic construct
SEVEFSHEYWMRHALTLAKRARDEREVPVGAVLVLNNRVIGVGWNRAIGLHDPTAHAEIMALRQGGLVMQNYRLTDATLYVTFEPCVMCAGAMVHSRIGRVVFGVRNSKRGAAGSLMNVLNYPGMSHCVGITEGILVDECAALLCDFYRMPRQVLDAQKKAQSSINSGGSSGGSSGSETQGTSESATPGSSGGGSSGSAKNTITKTLQLRIVRPYNSAEVEKIVADEKNNREKIALEKNKDKVKEACSKHLKVASYCTTQVERNACLFCKARKLDDKFYQKLRGQFPDAVFWQELGEIFRQLQKQAAEIYNQSLIELYYEIFIKGKGITNASRVEHYLSDVCYTRAAELFKNAAIASGLRSKVRSNFRLKELKNMKSGLPTTKSDNFPIPLVKQKGGQYTGFEISSHNDDFIIKIPFGRWQVKKEINKYRPWEKFDFEQVRKSPKPISLLLSTQRRKRNKGWSKDEGTEAEIRKVMNGDYQTSYIEVKRGSKIGEKSAWMLSLSIDVPKIDKGVDPSIIGGIDVGVKSPLVCAINNAFSRYSIGDNDLFRFNKKMFARRRILLKKNRHQRAGHGAKNKLKPITVLTEKSGRFRKKLIERWACEIADFFIKNKVGTVQMENLESMKRKEDSYFNIRLRGFWPYAEMQNKIEFKLKQYGIEIRKVAPNNTSKTCSKCGHLNNYFNFEYRKKNKFPHFKCEKCNFKENADYNAALNISNPKLKSAKEEP

SEQ ID NO: 2702 - protein, 726 aa, synthetic construct
SEVVFSHEYWMRHALTLAKRARDEREVPVGAILVLNDRVIGEGWNRAIGLHDPTAHAEIMALRQGGLVMQNYRLIDATLYVTFEPCVMCAGAMIHSRIGRVVFGVRNSKHGAAGSLMNVLNYPGMNHRVEITEGILADECAALLCDFYRMPRQVFNARKKARSNINSGGSSGGSSGSETLGTREGATPKSSGGSSAGSTKNTITKTLKLRIVRPYNSAEVEKIVADEKNSREKIALEKNKDKVKEACSEHLKVAAYCTTQVERNACLFCKARKLDDRFYQKLRGQFPDAVFWQEIGEIFRQLQKQAAEIYNQSLIELYYEIFIKGKGFANASSVEHYLSDVCYTRAAELFKNAAIASGLRGKIKSNFRLKELRNMKSGLPTTKSDNFPIPLVRQKGGQYTGFEISNHNGDFIIKIPFGRWQVKKEICKHRPWEKFDFEQVRKSPKPISLLLSTQRRKRNKGWGKDEGTEAEIRKVMNGDYQTSYIEVKRGSKIGEKSAWMLNLSIDVPKIDKGVDPSIIGGIDVGVKSPLVCAINNAFSRYSISDNDLYRFNKKMFARRRILLKKSRHKRAGHGAKNKLKPITILTEKSRRFRKKLIERWACEIADFFVKNKVGTVQMENLEGMKRKEDSYFNIRLRGFWPYAEMQNKIEFKLKQYGIKVRMVAPNNTSKTCSKCGHLNNYFSFEYRKKNKFPHFKCKKCNFKENADYNAALNISNPKLKSTKEEP

SEQ ID NO: 2703 - protein, 726 aa, synthetic construct
SEDEFSHEYWMRHALTLAKRARDGREVPVGAVLVLNNRVIGEGWNRAIGLHDPTAHAEIMALRQGGLVMQNYRLIDATLYVTFEPCVMCAGAMVHSRIGRVVFGVRNSKRGAAGSLMNVLDYPGMGHRVEITEGILADECAGLLCDFYCMPRQVFNAQKRAQSSINSGGSSGGSSGGDTPGASESVTPKSSGGSSTGSTKNTITKTLKLRIVRPYNSAEVEKIVADEKNNREKIALEKNKDKVKEACSEHLKMAAYCTTRVERNACLFCKARKLDDRFYQKLRGQFPDAVFWQEIGEIFRQLQKQAAEIYNQSLIELYYEIFIKGKGFANASSVEHYLSGVCYTRAAELFKNAAIASGLRGKVKSNFRLKELKNMKSGLPTTKSDNFPIPLVKQKGGQYTGFEISSHNSDFIIKIPFGRWQEKKEIDKYRPWEKFDFEQVRKNPKPISLLLSTQRRKGNKGWSKDEGTEAEIRKVMNGDYQTSYIEVKRGSKIGEKSAWMLNLSIDVPKIDKGVDPSIIGGIDVGVKSPLVCAINNALSRYSISDNDLFRFNKKMFARRRILLKKNRHRRAGHGAKNKLKPIAVLAEKSEGFRKKLIERWACEVADFFIKNKVGTVQMENLESMKRREDSYFNIRLRGFWPYAEMQNKIEFKLRQYGIEIRKVAPNNTSKTCSKCGHLNNYFDFEYRKKNKFPHFKCEKCNFKENADYNAALNISNPKLKSTKEGP

SEQ ID NO: 2704 - protein, 726 aa, synthetic construct
SEDEFSHEYWMRHALTLAKRARDGREVPVGAVLVLNNRVIGEGWNRAISLHDPTAHAEIMALRQGGLVMQNYRLIDATLYVTFEPCVMCAGAMVHSRIGRVVFGVRNGKRGAAGSLMNVLDYPGMGHRVEITEGILADECAALLCDFYCMPRQVFNAQKRAQSSINSGGSSGGNSGSETPGTSESATPGSSGGGSSGSAKNTITKTLQLRIIRPYNSAEVEKIVADEKNSREKIALEKNKDKVKEACSEHLKVAAYCTTQVERNACLFCKARKLDDRFYQKLRGRYPDAVFWQEIGEIFRQLQKQAAEIYNQSLIELYYEIFIKGKGFANASSVEHYLSDVCYTRAAELFKNAAIASGLRGKVKSNFRLKELKNMKSGLPTTKSDNFPIPLVKQKGGQYTGFEISSHNDDFIIKIPFGRWQVKKEIDKYRPWEKFDFEQVRKSPKPISLLLSTQRRKRNKGWSKDEGTEAEIRKVMNGDYQTSYIEVKRGSKIGEKSAWMLNLSIDVPKIDKGVDPSIIGGIDVGVKSPLVCAIDNAFSRYSISDNDLYHFNKKMFAKRRILLKKNRHKRAGHGAKNKLKPISILTEKSERFRKKLIERWACEIADFFIKNKVGTVQMENLESMKRREDSYFNTRLRGFWPYAEMQNKIEFKLKQYGIEIRKVAPNNTSKTCSKCGHLNNYFNFEYRKKNKFPHFKCEKCNFKENADYNAALNISNPRLKSTKEEP

SEQ ID NO: 2705 - protein, 726 aa, synthetic construct
SEVEFSHEYWMRRALALAKRARDEREVPVGAVLVLNNRVIGVGWNRAVGLHDPTAHAEIMALRQGGLVMQNYRLFDATLYVTFEPCVMCAGAMIHSRIGRVVFGVRNSKHGAAGSLVNVLNYPGMNHRVEITEGILVDECAALLCDFYRMPRQVFNAQKKAQSTINSGGSSGGSSGSETPGTSESPTPESSGGSPGGSAKNTITKTLKLRIVRPYNSAEVEKIVADEKNNREKIALEKNKDKVKEACSKHLKVASYCTTQVERNACLFCKARKLDDKFYQRLRGQFPDAVFWQELGEIFRQLQKQAAEIYNQSLIELYYEIFIKGKGFANANSVEHYLSDVCYTRAAELFKNAAIASGLRGKVKSNFRLKELKNMRSGLPTTKSDNFPIPLVRQKGGQYTGFEISSHNDDFIIKIPFGRWQVKKEIDKYRPWEKFDFEQVRKSPKPISLLLSTQRRKRNKGWSKDEGTEAEIRKVMNGGYQTSYIEVKRGSKTGEKSAWMLNLSIDVPKIDKGVDLNIIGGIDVGVKSPLVCAINNAFSRYSISDNDLFHFNKKMFARRRILLKKNRHKRAGHGAKNKLKPLTILTGKSKRFRKKLIERWACEIAGFFIKNKVGTVQMENLENMKRREDSYFNIRLRGFWPYAEMQNKIEFKLKQYGIEIRKVAPNNTSKTCSRCGHLNNYFNFEYRKRNKFPHFKCEKCNFKENADYNAALNISNPKLKSPKEEP

SEQ ID NO: 2706 - protein, 726 aa, synthetic construct
SEVEFSHEYWMRHALTLAKRARDEREVPVGAILVLNNRVIGEGWNRAIGLHDPTAHAEIMALRQGGLVMQNYRLIDATLYVTFEPCVMCAGAMIHSRIGRVVFGVRNSKRGAAGSLTNVLNYPGMSHRVEITEGILADECAALLCDFYRMPRQVFNARKKAQSNINPGGSSGGSSGSETPGTSESATPGSSGGSSGGSAKNTITKTLKLRIVRPYNSAEVEKIVADEKNNREKIALEKNKGKVKEACSEHLKVAAYCTTQVERNACLFCKARKLDDKFYQELRGQFPDAVFWQEIGEIFRQLQKQAAEIYNQSLIELYYEIFIKGKGFANASSVEHYLSDVCYTRAAELFKNAAIASGLRGKVKSNFRLKELRNMKSGLPTTKSDNFPIPLVRQKGGQYTGFKISSHNGDFIIKIPFGRWQVKKEIDKYRPWEKFDFEQVRKSPKPISLLLSTQRRKRNRGWGKDEGTEAEIKRVMNGDYQTSYIEVKRGSKIGEKSAWMLNLSIDVPKIDKGVDPRIIGGIDVGVKSPLVCAINNAFSRYSVSDNDLFHFNKKMFARRRILLKKNRHKRAGHGAKNKLEPITILTERSVRFRKKLIERWACEIADFFIKNKVGTVQMENLESMKGKEDSYFNIRLRGFWPYAEMQNKIEFKLKQYGIEIRKVAPNNTSKTCSKCGHLNSYFSFEYRKKNKFPHFKCEKCNFKEDADYNAALNISNPKLKSTKEEP

SEQ ID NO: 2707 - protein, 726 aa, synthetic construct
SEVEFSHEYWMRHALTLAKRARDEREVPVGAILVLNNRVIGEGWNRAIGLHDPTAHAEIMALRQGGLVMQNYRLIDATLYVTFEPCVMCAGAMIHSRIGRVVFGVRNSKHGAAGSLVNVLNYPGMNHRVEITEGILADECAALLCDFYRMPRQVFNARKKAQSSISSGGSSGGSSGSETPGASESVTPKSSVGSSAGSAKNTITKTLQLRIVRPYNSAEVEKIVADEKNNREKIALEKNKDKVKEACSKHLKVASYCTTQVERNACPFCKARKLDDKFYQKLRGQFPDAVFWQELGEILRQLQKQAAEIYNQSLIELYYEIFIKGKGFANASSVEHYLSDVCYTRAAELFKNAAIASGLRGKVKSNFRLKELRNMKSGLPTTKSDNFPIPLVRQKGGQYTGFEISNHNGDFIIKIPFGRWQVKKEVNKHRPWEKFDFEQVRKSPKPISLLLSTQRRKRNKSWSKDEGTEAEIRKVMNGDYQTSYIEVKRGSKIGEKSAWMLNLSIDVPKIDKGVDPSIVGGIDVGVKSPLVCAIDNALSRYSISDNDLFHFNKKMFARRRILLKKNGHRRAGHGAKNKLKPISILTEKSKRFRKKLIERWACEIADFFIKNKVGTVQMENLESMKRKEDSYFNIRLRGFWPYAEMQNKIEFKLKQYGIEIRKVAPNNTSKTCSKCGHLNSYFNFEYRRKNKFPHFKCEKCNFRENADYNAALNISNPKLKSTKGEP

SEQ ID NO: 2708 - protein, 726 aa, synthetic construct
SEVEFSHEYWMRHALTLAKRARDEREVPVGAVLVLNNRVIGEGWNRAIGLHDPTAHAEIMALRQGGLVMQNYRLIDATLYVTFEPCVMCAGAMIHSRIGRVVFGVRNSKHGAAGSLVNVLNYPGMNHRVEITEGILADECAALLCDFYRMPRQVFNARKKAQSSINPSGLSGGSSGSVTPGTSESATPESSGGGSSGSAKNTITKTLQLRIVRPYNSAEVEKIVADEKNNREKIALEKNKDKVREACSKHLKVASYCTTQVERNACPFCKARKLDDKFYQKLRGQFPDAVFWQELGEILRQLQKQAAEIYNQSLIELYYEIFIKGRGFANASSVEHYLSDVCYTRAAELFRNAAIASGLRNKIKSNFRLKELRNMKSGLPTTKSDNFPIPLVRQKGGQYTGFEISNHNDDFIIKIPFGRWQVKEEIDKYRPWEKFDFEQVRKSPKPISLLLSTQRRKRNKGWSKDEGTEAEIRKVMNGDYQTSYIEVKRGSKIGEKSAWMLNLSIDVPKIDKGVDPSIIGGIDVGVKSPLVCAINNAFCRYSISDNDLFHFNKKMFARRRILLKKSRHKRAGHGAKNKLKPISILTEKSKRFRKKLIERWACEIADFFIKNKVGTVQMENLESMKRKEDSYFNIRLRGFWPYAEMQSKIEFKLKQYGIKIRKVAPNNTSKTCSKCGHLNNYFNFEFRKKNKFPHFKCEKCNFKEDADYNAALNISNPKLKSTKEEP

SEQ ID NO: 2709 - protein, 726 aa, synthetic construct
SEDEFSHEYWMRHALTLAKRARDGREVPVGAVLVLNNRVIGEGWNRTTGLHDPTAHAEIMALRQGGLVMQNHRLVDATLYVTFEPCVMCAGAMIHSRIGRVVFGVRNSKRGAAGSLTNVLNYPGMNHRVEITEGILVDECAALLCDFYRMPRQVFNAQKKAQSTINSGGSSGGSSGSETPGTSESPTPESSGGSPGGSAKNTITKTLKLRIVRPYNSAEVEKIVADEKNSREKIALEKNKDKVKEACSKHLKVAAYCTTQVERNACLFCKARKLDDKFYQKLRGQFPDAVFWQEIGEIFRQLQKQAAEIYNQSLIELYYEIFIKGKGFANASSVEHYLSDVCYTRAAELFKNAAIASGLRGKVKSNFRLKELKNMKSGLPTTKSDNFPIPLVKQKGGQYTGFEISSHNDDFIIRIPFGRWQVKEEIDKYRPWEKFDFEQVRKNPKPISLLLSTQRRKRNKGWSKDEGTEAEIRKVMNGDYQTSYIEVKRGSKIGEKSAWMLNLSIDVPKIDKGVDPSIIGGIDVGVKSPLVCAINNAFSRYSISDNDLFRFNKKMFARRRILLKKNRHKRAGHGAKNKLKPISILTGKSERFRKKLIERWACEIADFFIKNKVGTVQMENLESMKRKEDSYFNIRLRGFWPYAEMQNKIEFKLKQYGIEIRKVAPNNTSKTCSKCGHLNNYFSFEYRKKNKFPHFKCEKCNFKENADYNAALNISNPKLKSTKEEP

SEQ ID NO: 2710 - protein, 726 aa, synthetic construct
SEVEFSHEYWMRHALILAKRARDEREVPVGAVLVLNNRVIGVGWNRAVGLHDPTAHAEIMALRQGGLVMQNYRLIEATLYVTFEPCIMCAGAMIHSRIGRVVFGVRNSKRGAAGSLMNVLNYPGMSHRVEITEGILADECAALLCDYYRMPRQVFNARKKAQSSINSGGSSDSGSGSETSGTCESVTPESSGGSSGGSAKNTITKTLKLRIVRPYNSAEVEKIVADEKNNREKIALEKNKGKVKEACSRHLEVAAYCTTQVERNACLFCKARKLDDKFYQKLRGQFPDAVFWQELGEIFRQLQKQAAEIYNQSLIELYYEIFIKGKGFANASSVEHYLSDVCYTRAAELFKNAAIASGLRGKVKSNFRLKELKNMKSGLPTTKSDNFPIPLVKQKGGQYTGFEISSHNDDFVIKIPFGRWQVKKEIDKYRPWEKFDFEQVRKGPKPISLLLSTQRRKRNKGWSKDEGTEAEIRKVMNGDYQTSYIEVKRGSKIGEKSAWMLNLSIDVPKIDKGVDPSIIGGIDVGVRSPLVCAIDNAFSRYSISDNDLFHFNKKMFARRRILLKKNRHKRAGHGAKNKLKPISILTEKSKRFRKKLIERWACEITDFFIKNKVGTVQMENLESMKRKEDSYFNIRLRGFWPYAEMQNRIELKLKQYGIEIRRVAPNNTSRTCSKCGHLNNYFNFEYRKKSKFPHFKCEKCNFREDADYNAALNISNPKLKSTKEEP

SEQ ID NO: 2711 - protein, 726 aa, synthetic construct
SEVEFSHEYWMRHALTLAKRARDEREVPVGAVLVLNNRVIGEGWNRAIGLHDPTAHAEIMALRQGGLVMQNYRLIDATLYVTFEPCVMCAGAMIHSRIGRVVFGVRNSKRGAAGSLMNVLNYPGMNHRVEITGGILTDECAALLCDFYRMPHQVLNAQKKAQSSINSGGSSGGSSGSETPGTGGSATPEGSGGISGGFAKSTITKTLKLRIVRPYNSAEVEKIVADEKSNREKIALEKNKGKVKEACSKHLKVATYCTTQVERNACLFCKARKLDDKFYQKLRGQFPDAVFWQEIGEIFRQLQKQAAEIYNQSLIELYYEIFIKGKGFANTSSVEHYLSDVCYTRAAELFKNAAIASGLRGKVKSNFRLKELRNMKSGLPTTKSDNFPIPLVRQKGGQYTGFEISNHNGDFIIKIPFGRWQVKKEINKHRPWEKFDFEQVRKSPKPISLLLSTQRRKGNKGWSKDEGTEAEIRRVMNGDYQTSYIEVKRGSKIGEKSAWMLNLSIDVPKIDKGVDPSITGGIDVGVKSPLVCAINNALSRYSISDNDLFHFNKKMFARRRILLRKNRHKRAGHGARNKLKPVTVLTEKSGRFRKKLIERWACEIADFFIKNKVGTVQMENLESMKRKEDSYFNIRLRGFWPYAEMQNKIEFKLKQYGIKIRKVAPNNTSKTCSKCGHLNNYFSFEYRKKNKFPHFKCEKCNFKEDADYNAALNISNPKLKSTKEEP

SEQ ID NO: 2712 - protein, 726 aa, synthetic construct
SEVEFSHEYWMRHALTLAKRARDEREVPVGAILVLNNRVIGEGWNRAIGLHDPTAHAEIMALRQGGLVMQNYRLIDATLYVTFEPCVMCAGAMIHSRIGRVVFGVRNSKHGAAGSLVNVLNYPGMNHRVEITEGILADECAALLCDFYRMPRQVFNARKKAQSSINPSGSSGGSSGSVTPGTSESAAPESSGGGFGGSAKNTITKTLQLRIVRPYNSAEVEKIVADEKNNREKIALEKNKDKVKEACSKHLKVASYCTTQVERNACPFCKARKLDDKFYQKLRGQFPDAVFWQELGEIFRQLQKQAAEIYNQSLIELYYVIFIKGKGLANASSVEHYLSDVCYTRAAELFKNAAIASGLRGKVKSNFKLKELKSMKSGLPSTKSDNFPIPLVKQRGGQYTGFEISSHNDDFIIKIPFGRWQAKKEIDKYRPWEKFDFEQVRKSPKPISLLLSTQRRKRNRGWSKDEGTEAEIRKVMNGDYQTSYIEVKRGSKIGEKSAWMLNLSIDVPKIDKGVDPSIIGGIDVGVKSPLVCAINNAFSRYSISDNDLFRFNKKMFARRRILLGKNRHKRAGHGVKNKLKPITMLTEKSGRFRKKLIERWACEIADFFIKNKVGTVQMENLESMKRKEDSYFNIRLRGFWPYAEMQDKIEFKLKQYGIEIRKVAPNNTSKTCSRCGHLNNYFNFEYRRKNKFPHFKCEKCNFKENADYNAALNISNPKLKSTKEEP

SEQ ID NO: 2713 - protein, 726 aa, synthetic construct
SEVEFSHEYWMRHALTLARRARDEREVPVGAILVLNNRVIGEGWNRAIGLHDPTAHAEIMALHQGGLVMQNYRLTDATLYVTFEPCVMCAGAMIHSRIGRVVFGARNSKRGAAGSLMNVLSYPGMNHRVEITEGILADECAALLCDFYRMPRRVFNAQKKAQSSINSGGSSGGGSGSDTPSTSESTTPESSGASSGGPAKNTITKTLKLRIVRPYNSAEVEKIVTDEKNNREKIALEKNKDKVKEACSQHLKMASYCTTQVERNACLFCKARKLDDKFYQKLRGQFPDAVFWQELGEIFRQLQKQAAEIYNQSLIELYYEIFIKGKGFANASSVEHYLSGVCYTRAAELFKNAAIASGLRGKVKSNFRLKELKNMKSGLPTTKSDNFPIPLVKQKGGQYTGFEISSHNDDFIIKIPFGRWQVKKEIDKYRPWEKFDFEQVRKSPKPISLLLSTQRRKRNKGWSKDVGTEAEIRKVMNGDYQTSYIEVKRGSKIGEKSAWMLNLSIDVPKIDKGVDPSVIGGIDVGVKSPLVCAINNAFSRYSISDNDLFRFNKKMFARRRILLKKNRHKRAGHGAKNKLKPITILTEKSRRFRKKLIERWACEIADFFIKNKVGTVQMENLECMKRKEDSYFNIRLRGFWPYAEMQNKIEFKLKQYGIKIRKVAPNNTSKTCSKCGHLNNYFSFEYRKKNKFPHFKCEKCNFKEDADYNAALNISNPKLKSTKEEP

SEQ ID NO: 2714 - protein, 726 aa, synthetic construct
SEVEFSHEYWMRHALTLAKRARDEREVPVGAILVLNNRVIGEGWNRAIGLHDPTAHAEIMALHQGGLVMQNYRLIDATLYVTFEPCVMCAGAMIHSRIGRVVFGARNSKRGAAGSLMNVLSYPGMNHRVEITEGILADECAALLCDFYRMPRRVFNAQKKAQSSINSGGSSGGGSSSDTPSTSESTTPESSGGSSGGPAKNTITKTLKLRIVRPYNSAEVEKIVADEKNNREKTALEKNKDKVKEACSKHLKVAAYCTTQVERNACLFCKARKLDDKFYQKLRGQFPDAVFWQEVGEIFRQLQKQAAEIYNQSLIELYYEIFIKGKGFANASSVEHYLSDVCYTRAAELFKNAAIASGLRGKVKSNFRLKELKNMKSGLPTTKSDNFPIPLVKQKGGQYTGFEISNRNSDFIIKIPFGRWQVKKEINKYRPWEKFDFEQVRKSPKPISLLLSTQRRKRNKGWSKDEGTEAEIRKVMSGDYQTSYIEVKRGSKIGEKSAWTLSLSIDVPKIDKGVDPSIIGGIDVGVKSPLVCAINNALSRYSIGDNDLFHFNKKMFARRRILLKKNRHKRAGHGTRNKLKPITVLTEKSERFRKKLIERWACEIANFFVKNKVGTVQMENLESMKRREDSYFNIRLRGFWPYAEMQNKIEFKLKQYGIEIRKVAPNNTSKTCSKCGHLNNYFNFEYRKKNKFPYFKCEMCNFKEDADYNAALNISNPKLKSTKEEP

SEQ ID NO: 2715 - protein, 726 aa, synthetic construct
SENEFSHEYWMRHALTLAKRARDGREVPVGAVLVLNNRVIGEGWNRAIGLHDPTAHAEIMALRQGGLVMQNYRLIDATLYVTFEPCVMCAGAMVHSRIGRVVFGVRNSKRGAAGSLMNVLDYPGMGHRVEITEGILADECAALLCDFYCMPRQVFNAQKRAQSSINSGGSSDGGSGSETPGTSESATPESSGGSSGGSAKNTITKTLKLRIVRPYNSAEVEKIVADEKNNREKIALEKNKDKVKEACSKHLKVASYCTTQVERNACLFCKARRLDDKFYRKLRGQFPDAVFWQEIGEIFRQLQKQAAEIYNQSLVELYYEILIKGKGIANASSVEHYLSDVCYTRAAELFKNAAIASGLRNKIKSNFRLKELRNMKSGLPTTKSDNFPIPLVKQKGGQYTGFEISSHNSDFIIKIPFGRWQVKEEIDKFRPWEKFDFEQVRKSPKPISLLLSTQRRKKNKGWSKDEGTEAEIRRVMNGDYQTSYIEVKRGSKIGEKGAWMLNLSIDVPKIDKGVDPSIIGGIDVGVKSPLVCAINNAFSRYSISDNELFHFNKKMFARRRILLKKNRHKRAGHGAKNKLKPISVLTEKSGRFRKKLIERWACEITDFFIKNKVGTVQMENLGSMKRREDSYFNIRLRGFWPYAEMQNKIEFKLKQYGIEIRKVAPDNTSKTCSKCGHLNNYFNFEYRKKNKFPHFKCEKCNFKEDADYNAALNISNPKLKGTKEEP

SEQ ID NO: 2716 - protein, 726 aa, synthetic construct; identical to SEQ ID NO: 2438

SEQ ID NO: 2717 - protein, 726 aa, synthetic construct
SEVEFSHEYWMRHALTLAKRARDGREVPVGAVLVLNNRVIGEGWNRAIGLHDPTAHAEIMALRQGGLVMQNYRLIDATLYVTFEPCVMCAGAMVHSRIGRVVFGVRNSKRGAAGSLMNVLDYPGMGHRVEITEGILADECAALLCDFYCMPRQVFNAQKRAQSSINSGGSSGGSSGSETPGTSESATPESSGGGSSGSAKSTITKTLQLRIVRPYNSAEVEKIVADEKNNREKIALEKNKDKVKEACSKHLKVASYCTTQVERNACLFCKARKLDDKFYQKLRGQFPDAVFWQELGEIFRQLQKQAAEIYNQSLVELYYEIFIKGKGIANASSVEHYLSDVCYTRAAELFKNAAIASGLRNKIKSNFRLKELRNMKSGLPTTKSDNFPIPLVRQKGGQYTGFEISNHNGDFIIKIPFGRWQVKKEIDKYRPWEKFDFEQVRKSPKPISLLLSTQRRKRNKGWSKDEGTEAEIKRVMNGDYQISYIEVKRGSKIGEKSAWMLSLSVDVPKIDKGVDPSIIGGIDVGVKSPLVCAINNALSRYSISDNDLFHFNKKMFARRRILLRNNRHKRAGHGAKSKLKPITILTEKGERFRKKLIERWACEIANFFIKNKVGTVQMENLESMKRKEDSYFNARLRGFWPYAEMQNKIEFKLKQYGIEIRKVAPNNTSKTCSRCGHLNNYFNFEYRRKNKFPHFKCEKCNFKENADYNAALNISDPKLKSTKEEP

SEQ ID NO: 2718 - protein, 726 aa, synthetic construct
SEVEFSHEYWMRHALTLAKRARDEREVPVGAILVLNNRVIGEGWNRAIGLHDPTAHAEIMALRQGGLVMQNYRLIDATLYVTFEPCVMCAGAMIHSRIGRVVFGVRNSKHGAAGSLVNVLNYPGMNHRVEITEGILADECAALLCDFYRMPRQVFNARKKAQSSINPSGSSGGSSGSVTPGTSESATPESSGGGFGGSAKNTITKTLQLRIVRPYNSAEVEKIVADEKNNREKIALEKNKDKVKEACSKHLKVAAYCTTQVERNACLFCKARKLDDKFYQKLRGQFPDAVFWQEIGEIFRQLQKQAAEIYNQSLIELYYEILIKGKGFANASSVEHYLSDVCYTRAAELFKNAAIASGLRGKVKSNFRLKELKNMRSGLPTTKSDNFPIPLVKQKGGQYAGFEISSHNDDFIIKIPFGRWQVKKEIDKYRPWEKFDFEQVRKSPKPISLLLSTQRRKRNKGWSKDEGTEAEIRKVMNGDYQTSYIEVKRGSKTGEKSAWMLNLSIDVPKIDKGVDPCIIGGIDVGVKSPLVCAINNAFSRYSISDNDLFHFNKKMFARRRILLKENGHKRAGHGAKNKLKPITIMTEKSKRFRKKLIERWACEIADFFIKNKVGTVQMENLESMKRKEDSYFNIRLRGFWPYAEMQNKIEFKLRQYGIEIRKVAPNNTSRTCSKCGHLNNYFNFEYRKKNKFPHFKCEKCNFKENADYNAALNISNPKLKSTKEEP

SEQ ID NO: 2719 - protein, 726 aa, synthetic construct
SEVEFSHEYWMRHALTLAKRARDEREVPVGAVLVLNNRVIGEGWNRTTGLHDPTAHAEIMALRQGGLVMQNHRLVDATLYVTFEPCVMCAGAMIHSRIGRVVFGVRNGKRGAAGSLTNVLNHPGMNHRVEITGGILADECAALLCDFYRMPRQVFNAQKKAQSTINSGGSSGGSSGSETPGTSESPTPESSGGSPGGSAKNTITKTLKLRIVRPYNSAEVEKIVADEKNNREKIALEKNKDKVKEACSKHLKVAAYCTTRVERNACLFCKARKLDDKFYQKLRGQFPDAVFWQEIGEIFRQLQKQAAEIYNQSLIELYYEIFIKGKGITNASRVEHYLSDVCYTRAAELFKNAAIASGLRSKVRSNFRLKELKNMKSGLPTTKSDNFPIPLVKQKGGQYAGFEISSHNSDFIIKIPFGRWQVKEEIDKYRPWEKFDFEQVRKSPKPISLLLSTQRRKKNKGWSKDEGTEAEIRRVMNGDYQTSYIEVKRGSKIGEKSAWMLNLSIDVPKIDKGVDPSIIGGIDVGVKSPLVCAVNNSFSRYSICDNDLFRFNKKMFARRRILLKKNRHKRAGHGAKNKLKPITILTKKSERFRKKLIERWACEVADFFIKNRVGTVQMENLESMKRKEDSYFNIRLRGFWPYAEMQNRIEFKLKQYGIEIRRVAPNNTSRTCSKCGHLNNYFNFEYRKKNKFPHFKCEKCNFREDADYNAALNISNPKLKSTKEEP

SEQ ID NO: 2720 - protein, 726 aa, synthetic construct
SEDEFSHEHWMRHALTLAKRARDEREVPVGAVLVLSNRVIGAGWNRTTGLHDPTAHAEIMALRQGGLVMQNYRLIDATLYVTFEPCIMCAGAMIHSRIGRVVFGVRNSKRGAAGSLMNVLNYPGMNHRVEITEGILADECAALLCDYYRMPRQVFNARKKAQSSINSGGSSDGGSGSETPGTSESATPESSGGSSGGSAKNTITKTLKLRIVRPYNSAEVEKIVADEKNNREKIALEMNKDKVKEACSKHLKVASYCTTQVERNACPFCKARKLDDKFYQKLRGQFPDAVFWQELGEILRQLQKQAAEIYNQSLIELYYEIFIKGRGFANASSVEHYLSDVCYTRAAGLFKNAAIASGLRNKIKSNFRLKELKNMKSGLPTTKSDNFPIPLVKQKGGQYTGFEISSHNDDFIIKIPFGRWQAKKEIDKYRPWEKFDFEQVRKSPKPISLLLSTQRRKKNKGWSKDEGTEAEIRRVMNGDYQTSYIEVKRGSKIGEKSAWMLNLSIDVPKIDKGVNPSIIGGIDVGVKSPLVCAINDSSSRYSICDNDLFRFNKKMFARRRILLKKNRHKRAGHGAKNKLKPISILTERSKRFRKKLIERWACEIADFFIKNKVGTVQMENLESMKRKEDSYFNIRLRGFWPYAEMQNKIEFKLKQYGIEIRKVAPNNTSKTCSKCGHLNNYFNFEYRKMNKFPHFKCEKCNFKENADYNAALNISNPKLKSTKEEP

SEQ ID NO: 2721 - protein, 726 aa, synthetic construct
SEVEFSHEYWMRHALSLAKRARDEREVPVGAVLVLNNRIIGEGWNRAIGQHDPTAHAEIMALRQGGLVMQNNRLTDATLYVTFEPCVMCAGAMVHSRIGRVVFGVRNSKRGAAGSLMNVLNYPGVNHCVEITEGILADECAALLCDFYCMPRQVFNARKKAQSSINPGGPSGGSSGSKTPGTSESATPEGSGGSSGGSAKNTITKTLKLRIVRPYNSAEVEKIVADEKNNREKTALEKNKDKVKEACSKHLKVAAYCTTQVERNACLFCKARKLDDKFYQKLRGQFPDAVFWQEIGEIFRQLQKQAAEIYNQSLIELYYEIFIKGKGFANASSVEHYLSDVCYTRAAELFKNAAIASGLRGKVKSNFRLKELKNMKSGLPTTKSDNFPIPLVKQKGGQYTGFEISDHNSDFIIKIPFGRWQAKKEIDKYRPWEKFDFEQVRKSPKPISLLLSTQRRKKNKGWSKDEGTEAEIKKVMNGDYQTSYIEVKRGSKTGEKSAWMLNLSIEVPKIDKGVDPCIIGGIDVGVKSPLVCAINNAFSRYSISDNDLFHFNKKMFARRRILLKKNGHKRAGHGAKNKLRPITIMTEKSKRFRKKLIERWACEIADFFIKNKVGTVQMEDLESMKRKEDSYFNIRLRGFWPYAEMQNKIEFKLKQYGIKIRKVAPNNTSKTCGKCGHLNNYFNFEYRKKNKFPHFKCEKCNFKENADYNAALNISNPKLKSTKEEP

SEQ ID NO: 2722 - protein, 725 aa, synthetic construct
SEVEFSHEYWMRHALTLAKRARDEREVPVGAVLVLNNRVIGEGWNRAIGLHDPTAHAEIMALRQGGLVMQNYRLTDATLYVTFEPCVMCAGAMIHSRIGRVVFGVRNSKRGAAGSLMNVLNYPGMNHCVEITEGILVDECAALLCDFYRMPRQVLNAQKKAQSSISSGGSSGGSSGSETPGASGSVTPKSSGGSSAGSTKDTITKTLKLRIVRPYNSAEVEKIVADEKNSREKIALEKNKDKVKEACSEHLRVAAYCTTQVERNACLFCKARKLDDGFYQKLRGQFPDAVFWQEIGEIFRQLQKQAAEIYNQSLIELYYEIFIKGKGITNASRVEHYLSDVCYTRAAELFKNAAIASGLRSKVRSNFRLKELKNMRSGLPTTKSDNFPIPLVKQKGGQYTGFEISSHNSDFIIKIPFGRWVKKEIDKYRPWEKFDFEQVRKSPRPISLLLSTQRRKRNKGWSKDEGTEAEIRKVMNGDYQTSYIEVKRGSKIGEKSAWMLNLSIDVPKIDKGVDPSIIGGIDVGVKSPLVCAIDNALSRYSISDNDLFHFNKKMFARRRILLKKNRHRRAGHGAKNKLKPISILTEKSKRFRKKLIERWASEIANFFIKNKVGTVQMENLESMKRKEDSYFNIRLRGFWPYAEMQNKIEFKLKQYGIEIRKVAPDNTSKTCSKCGHLNNYFNFEYRKKNKFPHFKCEKCNFKEDADYNAALNISNPKLKSTKEEP

SEQ ID NO: 2723 - protein, 726 aa, synthetic construct
SEVEFSHEYWMRHALTLAKRARDEREVPVGAILVLNNRVIGEGWNRAIGLHDPTAHAEIMALRQGGLVMQNYRLIDATLYVTFEPCVMCAGAMIHSRIGRVVFGVRNSKHGAAGSLVNVLNYPGMNHRVEITEGILADECAALLCDFYRMPRQVFNARKKAQSSINPSGSSGGSSGSVTPGTSESPTPESSGGSSGGSAKSTITKTLKLRIVRPYNSAEVEKIVADEKNNREKIALEKNKGKVKEACSRHLEVAAYCTTQVERNACLFCKARKLDDKFYQKLRGQFPDAVFWQELGEIFRQLQRQAAEIYNQSLIELYYEIFIKGKGFANASSVEHYLSDVCYTRAAELFKNAAIASGLRGKVKSNFRLKELKNMKSGLPTTKSDNFPIPLVKQKGGQYTGFEISSRNDDFIIKIPFGRWQVRKEIDKYRPWEKFNFEQVRKSPKPISLLLSTQRRKRNKGWSKDEGTEAEIRKVMNGDYQTSYIEVKRGSKIGEKSAWMLSLSIDVPKIDKGVDPSIIGGIDVGVKSPLVCAINNAFNRYSISDNNLFHFNKKMFARRRILLKKNRHKRAGHGAKNKLKPISILTEKSKRFRKKLIERWACEIADFFIKNKVGTVQMENLESMKRKEDSYFNIRLRGFWPYAEMQNKIEFKLKQYGIEIRKVAPNNTSKTCSKCGHLNNYFNFEYRKMNKFPHFKCEKCNFKENADYNAALNISNPKLKSTKEEP

SEQ ID NO: 2724 - protein, 726 aa, synthetic construct
SEVEFSHEYWMRHALTLAKRARDEREVPVGAVLVLNNRVIGEGWNRAIGLHDPTAHAEIMALRQGGLVMQNYRLTDATLYVTFEPCVMCAGAMIHSRIGRVVFGVRNSKRGAAGSLMNVLNYPGMNHCVEITEGILADECAALLCDFYRMPRQVFNARRKAQSSINPGGSSGGSSGSETPGTSESPTPESSGGSSGGSAKNTITKTLRLRIVRPYNSAEVEKIVADEKNNREKIALEKNKDKVKEACGKHLKVASYCTTQVERNACLFCKARKLDDKFYQKLRGQFPDAVFWQELGEIFRQLQKQAAEIYNQSLIELYYEIFIKGKGFANASSVEHYLSDVCYTRAAELFKNAAIASGLRGKVKSNFKLKELKSMKSGLPSTKSDNFPIPLVKQKGGQYTGFEISSHNDDFIIKIPFGRWQVKEEIDKYRPWEKFDFEQVRRNPKPISLLLSTQRRKRNKGWSKDEGTEAEIRKVMNGDYQTSYIEVKRGSKIGEKSAWMLSLSIDVPKINKGVDPSIIGGIDVGVKSPLVCAINNASSRYSISDNDLFRFNKKMFARRRILLRKNRHKRAGHGARNKLKPITVLTEKSERFRKKLIERWACEIANFFIKNKVGTVQMENLESMKRREDSYFNIRLRGFWPYAEMQSKIEFKLKQYGIEVRRVAPNNTSKTCSKCGHLNNYFNFEFRKKNKFPHFKCEKCNSKEDADYNAALNISNPKLKSTKEEP

SEQ ID NO: 2725 - protein, 726 aa, synthetic construct
SEVEFSHEYWMRHALTLAKRARDEREVPVGAILVLNNRVIGEGWNRAIGLHDPTAHAEIMALRQGGLVMQNYRLIDATLYVTFEPCVMCAGAMIHSRIGRVVFGVRNNKRGAAGSLMNVLNYPGMNHRVEITEGILADECAALLCDFYRMPRQVFNAQKKAQSSTNPGGSSGGSSGSETPGTSESATPESPGGSSGGSAKNTITKTLKLRIVRPYNSAEVEKIVADEKNNREKIALEKNKDKVKEACSKHLKVAAYCTTQVERNACLFCKARRLDDKFYQKLRGQFPDAVFWQELGEIFRQLQKQAAEIYNQSLIELYYEIFIKGKGLANASSVEHYLSDVCYTRAAELFKNAAIASGLRGKVKSNFKLKELKSMKSGLPSTKSDNFPIPLVKQKGGQYTGFEISSHNDDFIIKIPFGRWRVKKEIDKYRPWEKFDFEQVRRSPRPISLLLSTQRRKRNKGWSKDEGTEAEIRKVMNGDYQTSYIEVKRGSKIGEKSAWMLNLSIDVPKIDKGVDPSIIGGIDVGVKSPLVCAIDNALSRYSISDNDLFHYNKKMFARRRILLKKNRHKRAGHGAKNKLRPISILTEKSERFRKKLIERWACEIANFFIKNRVGTVQMENLESMRRKEDSYFNIRLRGFWPYAEMQNKIEFKLKQYGIGIRKVAPNNTSKTCSKCGHLNNYFNFEYRKKNKFPHFKCEKCNFKENADYNAALNISNPKLKSTKEEP

SEQ ID NO: 2726 - protein, 726 aa, synthetic construct
SEVEFSHEYWMRRALTLAKCARDEREVPVGAVLVLNNRVIGVGWNRAVGLHDPTAHAEIMALRQGGLVMQNYRLVEATLYVTFEPCIMCAGAMIHSRIGRVVFGVRNSKRGAAGSLMNVLNHPGMNHRVEITEGILADECAALLCDYYRMPRQVFNARKKAQPSINSGGSSDGGSGSETPGASESATPKSSGGSSGGSAKNTITKTLKLRIVRPYNSAEVEKIVADEKNNRERIALEKNKDKVKEACSKHLKVASYCTTQVERNACLFCKARKLDDKFYQKLRGQFPDAVFWQEIGDIFRQLQKQAAEIYNQSLIELYYEIFIKGKGITNASSVEHYLSDVCYARAAELFKNAAIASGLRSKVKSNFRLKELKNMKSGLPTTKSVNFPIPLVKQKGGQYTGFEVSNHNSDFIIKIPFGRWQVKKEINKYRPWEMFDFEQVRKSPKPISLLLSTQRRKRNKGWSKDEGTEAEIRKVMNGDYQVSYIEVKRGSKIGEKSAWMLNLSIDVPKIDKGVDPSIIGGIDVGVKSPLVCAINNALSRYSISDNDLFHFNKKMFARRRILLKKNRHKRAGHGARNKLKPITVLTEKSERFRKKLIERWACEIANFFIKNKVGTVQMENLESMKRKEDSYFNNRLRGFWPYAEMQNKIELKLRQYGIEIRKVAPNNTSKTCGKCGHLNNYFNFEYRKKNKFPHFKCEKCNFKENADYNAALNISNPKLKSTKEEP

SEQ ID NO: 2727 - protein, 726 aa, synthetic construct
SEVEFSHEYWMRHALTLAKRARDEREVPVGAVLVLNNRVIGEGWNRTIGLHDPTAHAEIMALRQGGLVMQNYRLIDATLYVTFEPCVMCAGAMIHSRIGRVVFGVRNSKRGAAGSLMNVLNYPGINHCVEITEGILVDECAALLCDFYRMSRQVLNAQKKAQSSISSGGSSGGSSGSETPGASGSVTPKSSVGSSAGPTRNTITKTLKLRIVRPYNSAEVEKIVADEKDNREKIALEKNKDKVKEACSEHLKVAAYCTTQVERNACLFCKARKLDDKFYQKLRGQFPDAVFWQEIGEIFRQLQKQAAEIYNQSLIELYYEIFIKGKGFANASSVEHYLSDVCYTRAAGLFKNAAIASGLRGKVKSNFRLKELKNMKSGLPTTKSDNFPIPLVKQKGGQYTGFEISSHNDDFIIKIPFGRWQVKKEIDKYRPWEKFDFEQVRKSPKPISLLLSTQGRKKNKGWSGDEGTEAEVKKVMNGDYQISYIEVKRGSKIGEKSAWTLNLSIDVPKIDKGVDPSIIGGIDVGVKSPLVCAISNALSRYSINDNDLFHFNKKMFARRRILLKKSKHKRAGHGAKNKLKPITILTEKSRRFRKKLIERWACEIADFFIKNKVGTVQMENLESMKRKEDSYFNIRLRGFWPYAEMQNKIEFKLKQYGIVVRKVAPNNTSKTCSKCGHLNNYFNFEYRKKNKFPHFKCEKCNFKEDADYNAALNISNPKLKSTKGEP

SEQ ID NO: 2728 - protein, 726 aa, synthetic construct
SEVEFSHEYWMRHALTLAKRARDEREVPVGAVLVLNNRVIGEGWNRTTGLHDPTAHAEIMALRQGGLVMQNHRLVDATLYVTFEPCVMCAGAMIHSRIGRVVFGVRNSKRGAAGSLTNVLNYPGMNHRVEIMEGILVDECAALLCDFYRMPRQVFNAQKKAQSTINSGGSSGGSSGSETPGTSESPTPESSGGSPGGSAKNTITKTLKLRIVRPYNSAEVEKIVADEKNNREKIALEKNKDKVKEACSKHLKVAAYCTTQVERNACLFCKARKLDDKFYQKLRGQFPDAVFWQEIGEIFRQLQKQAAEIYNQSLIELYYEIFIKGKGFANASSVEHYLSDVCYTRAAELFKNAAIASGLRGKVKSNFRLKELKNMKSGLPTTKSDNFPIPLVKQKGGQYTGFEISSHNDDFIIKIPFGRWQVKKEIDKYRPWEKFDFEQVRKSPKPISLLLSTQRRKRNKGWGKDEGTEAEIKRVMNGDYQTSYIEVKRSSKIGEKSAWMLNLSIDVPKIDKGVDPRIIGGIDVGVKSPLVCAINNAFSRYSVSDNDLFHFNKKMFARRRILLKKNRHKRAGHGAKNKLKPITILTEKSVRFRKKLIERWACEIADFFIKNKVGTVQMENLESMKGKEDSYFNIRLRGFWPYAEMQNKIEFKLKQYGIEIRKVAPNNTSKTCSKCGHLNNYFNFEYRKKNKFPHFKCEKCYFKEDADYNAALNISNPKLRSTKEEP

SEQ ID NO: 2729 - protein, 726 aa, synthetic construct
SEVEFSHEYWMRHALTLAKRARDGREVPVGAVLVLNNRVIGEGWNRAIGLHDPTAHAEIMALRQGGLVMQNYRLIDATLYVTFEPCVMCAGAMIHSRIGRVVFGVRNSKHGAAGSLMNVLNYPGMNHRVEITEGILADECAGLLCDFYRMPRQVFSARKKAQSSINPGGSSGGSSGGKAPGTSESATLESSGGSSGGSAKNTITKALKLRIVRPYNSAEVEKIVADEKNNRERIALEKNKDKVKEACSKHLKVAAYCTTQVERNACLFCKARKLDDKFYQKLRGQFPDAVFWQEIGEIFRQLQKQAAEIYNQSLIELYYEIFIKGKGFANASSVEHYLSDVCYTRAAELFKNAAIASGLRGKVKSNFRLKELKNMKSGLPTTKSDNFPIPLVKQKGGQYAGFEISSHNDDFVIKIPFGRWQVKKEIDKYRPWEKFDFEQVRKSPKPISLLLSTQRRKRNKGWSKDEGTEAEIRKVMNGDYQTSYIEVKRGSKIGEKSAWMLNLSIDVPKIDKGVDPSIIGGIDVGVKSPLVCAINNALSRYSISDNDLFHFNKKMFARRRILLKKNGHKRAGHGAKNKLKPISILTEKSERFRKKLIEKWACEIADFFIKNKVGTVQMENLESMKRKEDSYFNIRLRGFWPYAEMQNKIEFKLKQYGIEVRKVAPNNTSKTCSKCGHLNNYFNFEYRKKNKFPHFKCEKCNFKENADYNAALNISNPKLKSTKEEP

SEQ ID NO: 2730 - protein, 726 aa, synthetic construct
SEVEFSHEYWMRHALTLAKRARDEREVPVGAVLVLNNRVIGEGWNRAIGLHDPTAHAEIMALRQGGLVMQNYRLIDATLYVTFEPCVMCAGAMIHSRIGRVVFGVRNNKHGAAGSLVNVLNCPGMNHHVEITEGILADECAALLCDFYRMPRRVFNAQKKAHSSINSGGSSGGSSGSVTPGTSESATPESSGGSSGGSAKNTITKTLKLRIVRPYNSAEVEKIVADEKNSREKIALEKNKDKVKEACSEHLKVAAYCTTQVERSACLFCKARKLDDKFYQKLRGQFPDAVFWQEIGEIFRQLQKQAAEIYNQSLIELYYEVFIKGKGFANASSVEHYLSDVCYTRAAELFKNAAIASGLRGKVKSNFRLKELKNMKSGLPTTKSDNFPIPLVKQKGGQYTGFEISSHNDDFIIKIPFGRWQVRKEIDKYRPWEKFNFEQVRKSPKPISLLLSTQRRKRNKGWSKDEGTEAEIRKVMNGDYQTSYIEVKRGSKMGEKSAWMLNLSIDVPKIDKGVDPSITGGIDVGVKSPLVCAINNAFSRYSISDNDLFRFNKKMFARRRILLKKNRHKRAGHGAKNKLKPISILTGKSERFRKKLIERWACEIADFFIKNKVGTVQMENLESMKRREDSYFNIRLRGFWPYAEMQNKIEFKLKQYGIEIRKVAPNNTSKTCSKCGHLNNYFNFEHRKKNKFPHFKCEKCNFKENADYNAALNISNPKLKSTKEEP

SEQ ID NO: 2731 - protein, 726 aa, synthetic construct
SEVEFSHEYWMRHALTLAKRARDGREVPVGAVLVLNNRVIGEGWNRAIGLHDPTAHAEIMALRQGGLVMQNYRLIDATLYVTFEPCVMCAGAMVHSRIGRVVFGVRNSKRGAAGSLMNVLNYPGMGHRVEITEGILVDECAALLCDFYRMPRQVLNAQKKAQSSISSGGSSGGSSGSETPGTSESATPESSGGSSGGSAKNTITKTLKLRIVRPYNSAEVEKIVADEKNNREKIALEKNKDKVKEACSKHLKVAAYCTTQVERNACPFCKARKLDDKFYQKLRGQFPDAVFWQEIGEIFRQLQKQAAEIYNQSLVELYYEIFIKGRGIANASSVEHYLSDVCYTRAAELFKNAAIASGLRNKIKSNFRLKELRNMKSGLPTTKSDNFPIPLVRQKGGQYTGFEISNHNSDFIIKIPFGRWQVKKEIDKYRPWEKFDFAQVRKSPKPISLLLSTQRRKRNRGWSKDEGTEAEIKKVMNGDYQTSYIEVKRGSKIGEKSAWMLNLSIDVPKIDKGVDPSIIGGIDVGVKSPLVCAINNAFSRYSISDNDLFHFNKKMFARRRILLKRNRHKRAGHGAKNKLKPITTLTEKSKRFRKKLIERWACEIADFFIKNKVGTVQMENLESMKRKEDSYFNIRLRGFWPYAEMQNKIEFKLRQYGIEIRKVAPNNTSKTCSKCGHLNNYFNFEYRKKNKFPHFKCEKCNFKENADYNAALNISNPKLKSTKEKP

SEQ ID NO: 2732 - protein, 726 aa, synthetic construct
SEVEFSHEYWMRHALTLAKRARDGREVPVGAVLVLNNRVIGEGWNRAIGLHDPTAHAEIMALRQGGLVMRNHRLIDATLYVTFEPCVMCAGAMVHSRIGRVVFGVRNSKRGAAGSLVNVLDYPGMDHRVEITEGILADECAALLCDFYRMPHQVFNAQKKAQSSINSGGSSDGSSGSVTPGPSESATPESSGGSSGSSAKNTITKTLQLRIVRPYNSAEVEKIVADEKNNREKIALEKNKDKVKEACSKHLKVASYCTTQVERNACPFCRARKLDDKFYQKLRGQFPDAVFWQELGEILRQLQKQAAEIYNQSLIELYYEIFIKGRGFANASSVEHYLSDVCYTRAAELFKNAAIASGLRGKVKSNFRLKELKNMRSGLPTTKSDNFPIPLVRQKGGQYTGFEISNHDGDFIIKIPFGRWQVKKEINKHRPWEKFDFEQVRKSPKPISLLLSTQRRKRNKGWSKDEGTEAEIRRVMNGDYQTSYIEVKRGSKIGEKSAWMLNLSIDVPKIDKGVDPSIIGGIDVGVKSPLVCAINNAFSRYSISDNDLFHFNKKMFARRRILLKKNRHRRAGHGAKSKLKPITILTEKGERFRKKLIERWACEIADFFVKNKVGTVQMENLESMKRKEDSYFNIRLRGFWPYAEMQSKIEFKLKQYGIVVRKVAPNNTSKTCSKCGHLNNYFNFEFRKKNKFPHFKCEKCSFKENADYNAALNISNPKLKSTKEKP

SEQ ID NO: 2733 - protein, 726 aa, synthetic construct
SEVEFSHEYWMRHALTLAKRARDEREVPVGAILVLNNRVIGEGWNRAIGLHDPTAHAEIMALRQGGLVMQNYRLIDATLYVTFEPCVMCAGAMIHSRIGRVVFGVRNSKRGAAGSLMNVLNYPGMNHCVEITEGILVDECAALLCDFYRMPRQVLNAQKKAQSSINSGGSSGGSSSSATPGTSESATPESSGGSSGSSAKNTITKTLKLRIVRPYNSAEVEKIVVDEKNNREKIALEKNKDKVKEACSKHLKVAAYCTTQVERNACLFCKARRLDDKFYQKLRGQFPDAVFWQEIGEIFRQLQKQAAEVYNQSLVELYYEIFIKGKGFANASSVEHYLSDVCYTRAAELFKNAAIASGLRGKVKSNFRLKELKNMKSGLPTTKSDNFPIPLVKQKGGQYTGFEISSHNDDFIIKIPFGRWQVKKEIDRYRPWEKFDFEQVRKSPKPISLLLSTQRRKRNKGWSKDEGTEAEIRKVMNGDYQTSYIEVKRGSKIGEKSAWMLNLSIDVPKIDKGVDPSIIGGIDVGVKSPLVCAINNALGRFSISDNDLFHFNKKMFARRRILLRKNRHKRAGHGAKNKLKPISILTEKSRRFRKKLIERWACEIADFFIKNKVGTVQMEDLESMKRRGDNYFNIKLRGFWPYAEMQNKIEFKLKQYGIEIRRVAPNNTSRTCSKCGHLNDYFNFEYRRKYKFPHFKCEKCNFKEDADYNAALNISNPKLKSTKEEP

SEQ ID NO: 2734 - protein, 726 aa, synthetic construct
SEVEFSHEYWMRHALTLAKRARDEREVPVGAVLVLNNRVIGEGWNRAIGLHDPTAHAEIMALRQGGLVMQNYRLTDATLYVTFEPCVMCAGAMIHSRIGRVVFGVRNSKRGAAGSLMNVLNYPGMNHCVEITEGILVYECAALLCDFYRMPRQVLNAQKKAQSSISSGGSSGGSSGSETPGASGSVTPKSSGGSSAGPTKDTITKTLKLRIVGPYNSAEVEKVVADEKNNREKIALEKNKDKVKEACSKHLKVAAYCTTQVERNACLFCKARKLDDKFYQKLRGQFPDAVFWQELGGIFRQLQKQAAEIYNQSLIELYYEIFIKGKGITNASRVEHYLSDVCYTRAAELFKNAAIASGLRSKVRSNFRLKELKNMKSGLPTTKSDNFPIPLVKQKGGQYTGFEISNHNDDFIIKIPFGRWQVKKEIDKYRPWEKFDFEQVRKSPKPISLLLSTQRRKRNKGWSKDEGTEAEIRKVMNGDYQTSYIEVKRGSKTGEKSAWMLNLSIDVPKIDKGVDPSIVGGIDVGVKSPLVCAINNASSRYSISDNDLFHFNKKMFARRRILLGKNRHKRAGHGVKNKLKPITILTEKSGRFRKKLIERWACEIADFFVKNKAGTVQMENLESMKRKEDSYFNIRLRGFWPYAEMQNKIEFKLKQYGIKVRKVAPNNTSKTCSKCGHLNNYFSFEYRKKNKFPHFKCEKCNFKENADYNAALNISNPKLKSTKEEH

SEQ ID NO: 2735 - protein, 726 aa, synthetic construct
SEDEFSHEYWMRHALTLAKRARDGREVPVGAVLVLNNRVIGEGWNRAIGLHDPTAHAEIMALRQGGLVMQNYRLIDATLYVTFEPCVMCAGAMVHSRIGRVVFGVRNSKRGAAGSLMNVLDYPGMGHRVEITEGILADECAALLCDFYCMPRQVFNAQKRAQSSINSGGSSGGSSGSETPGTSESATPEISGGGSSGSAKDTITKTLQLRIVRPYNSAEVEKIVADEKNNREKIALEKNKGKVKEACSKHLKVASYCTTQVERNACPFCKARKLDDKFYQKLRGQFPDAVFWQELGEILRQLQKQAAEIYNQSLIELYYEIFIKGKGFANASSVEHYLSDVCYTRAAELFKNAAIASGLRGKVKSNFRLKELRSMKSGLPTTKSDNFPIPLVRQKGGQYTGFEISNHNSDFIIKIPFGRWQAKKEIDKYRPWEKFDFEQVRKSPKPISLLLSTQRRKRNRGWSKDEGTEAEIRRVMNGDYQTSYIEVKRGSKIGEKSAWMLNLSIDVPKIDKGVDPSIIGGIDVGVKSPLVCAINNSSSRYSICDNDLFRFNKKMFARRRILLKKNRHKRAGHGAKNKLKPITILTKKSERFRKKLIERWVCEVADFFIKNKVGTVQMENLESMKRKEDSYFNIRLRGFWPYAEMQNRIELKLKQYGIEIRRVAPNNTSRTCSKCGHLNNYFDFEYRKKNKFPHFKCEKCNFKENADYNAALNISNPKLKGTKEEP

SEQ ID NO: 2736 - protein, 726 aa, synthetic construct
SEVEFSHEYWMRHALTLAKRARDEREVPVGAVLVLNSRVIGVGWNRAISLHDPTAHAEIMALRQGGLVMQNHRLIDATLYVTFEPCVMCAGAMVHSRIGRVVIGVRNSKRGAAGSLMNVLNYPGMNHRVEITEGILADECAALLCDFYHMPHQVFNAQRKAQSSINFGGSSGGSSGSGTPGTCEGATPESPGGSSGGSAKNTITKTLKLRIVRPYNSAEVEKIVADEKNNREKIALEKNKDKVKEACSKHLKVASYCTTQVERNACPFCKARKLDDKFYQKLRGQFPDAVFWQELGEILRQLQKQAAEIYNQSLIELYYEIFIKGRGFANASSVEHYLSDVCYTRAAELFKNAAIASGLRGKVKSNFRLKELKNMKSGLPTTKSDNFPIPLVKQKGGQYTGFEISSHNDDIIIKIPFGRWQVKKEIDKYRPWEKFDFEQVRKSPKPISLLLSTQRRKRNKGWSKDEGTEAEIRKVMNGDYQTSYIEVKRGSKIGEKSAWMLNLSIDVPKIDKGVDPSIIGGIDVGVKSPLVCAINNAFSRYSISDNDLFHFNKKMFARRRILLKKNRHKRAGHGAKNKLKPIFILTEKSKRFRKKLIEKWACEIADFFIKNKVGTVQMENLESMKRKEDSYFNIRLRGFWPYAEMQNKIEFKLKQYGIEIRKVAPNNTSKTCSKCGHLNNYFNFEYRKKNKFPHFKCEKCNFKENADYNAALNISNPELKSTKEEP

SEQ ID NO: 2737 - protein, 726 aa, synthetic construct
SEVEFSHEYWMRRALTLAKRARDEREVPVGAVLVLNNRVIGVGWNRAVGLHDPTAHAEIMALRQGGLVMQNYRLIEATLYVTFEPCIMCAGAMIHSRIGRVVFGVRNSKHGAAGSLVNVLNYPGMNHRVEITEGILADECAALLCDFYRMPRQVFNARKKAQSSINSGGSSGGSSGSETPGTSESATPKSSGGSSGGSAKNTITKALKLRIVRPYNSAEVEKIVADEKNNREKIALEKNKDKVKEACSKHLKVAAYCTTQVERNACLFCKARRLDDKFYQKLRGQFPDAVFWQEIGEILRQLQKQAAEIYNQSLVELYYEILIKGKGIANASSVEHYLSDVCYTRAAELFKNAAIASGLRNKIKSNFRLKELRNMKSGLPTTKSDNFPIPLVRQKGGQYTGFEISNHDGDFIIKIPFGRWQVKKEINKHRPWEKFDFEQVRKSPKPISLLLSTQRRKRNKGWSKDEGTEAEIRKVMNGDYQTSYIEVKRGSKIGEKSAWMLNLSIDVPKIDKGVDPSIIGGIDVGVKSPLVCAINNALSRYSISDNDLFHFNKKMFARRRILLRKNRHKRAGHGARNKLKPITVLTEKSERFRKKLIERWACEIANFFIKNKVGTVQMENLESMKRREDSYFNIRLRGFWPYAEMQSKIEFKLKQYGIKIRKVAPNNTSKTCSKCGHLNSYFNFEFRKKNKFPHFKCEKCNFKEDADYNAALNISNPKLKSTKEEP

SEQ ID NO: 2738 - protein, 726 aa, synthetic construct
NEVEFSHEYWMRHALTLAKRARDEREVPVGAVLVLNNRVIGEGWNRAIGLHDPTAHAEIMALRQGGLAMQNYRLVDATLYVTFEPCVLCAGAMVHSRIGRVVFGVRNSKRGAAGSLMNVLNHPGMNHRVEITGGILADECAALLCDFYRMPRQVFNAQKKARSNINSGGSSGGSSGSETLGTSESATPKSSGGSSGGSAKNTITKALKLRIVRPYNSAEVEKIVADEKNNRERIALEKNKDKVKEACSKHLKVAAYCTTQVERNACLFCKARKLDDKFYQKLRGQFPDAVFWQEIGEIFRQLQKQAAEIYNQSLIELYYEILIKGKGFANASSVEHYLSDVCYTRAAELFKNAAIASGLRGKVKSNFRLKELKNMRSGLPTTKSDNFPIPLVKQKGGQYAGFEISSHNDDFIIKIPFGRWQVKKEIDKYRPWEKFDFEQVRKSPKPISLLLSTRRRKRNKGWSKDEGTEAEIRKVMNGDYQTSYIEVKRGSKIGEKSAWMLNLSIDVPRIDKGVDPSIIGGIDVGVKSPLVCAINNAFGRYSISDNDLFHFNKKMFARRRILLKKNRHKRAGHGAKNKLKPITILTEKSKRFRKKLIERWACEIADFFIKNKVGTVQMENLESMKRKEDSYFNIRLRGFWPYAEMQDKIEFKLKQYGIEIRKVAPNNTSKTCSRCGHLNNYFNFEYRKKSKFPHFKCEKCNFKENADYNAALNISNPKLKSTKEEP

SEQ ID NO: 2739 - protein, 726 aa, synthetic construct
SEDEFSHEYWMRHALTLAKRARDEREVPVGAVLVLNNRVIGEGWNRAIGLHDPTAHAEIMALRQGGLVMQNYRLVDATLYVTFEPCVLCAGAMVHSRIGRVVFGVRNSKRGAAGSLMNVLNYPGMNHRVEITEGILADECAALLCDFYRMPRQVFNARKKARSNNNSGGSSGGSSGSETPGTSESPTPESPGGSSGGSAKNTITKTLKLRIVRPYNSAEVEKIVADEKNNREKIALEKNKDKVKEACSKHLKVAAYCTTQVERNACLFCKARKLDDKFYQKLRGQFPDAVFWQEISEIFRQLQKQAAEIYNQSLIELYYEILIKGKGITNASSVEHYLSDVCYTRAAELFKNAAIASGLRGKVKSNFRLKELKNMKSGLPTTKSDNFPIPLVKQKGGQYTGFEISSHNDDFIIKIPFGRWQVKKEIDKYRPWEKFDFEQVRKSPKPISLLLSTQRRKRNKGWSKDEGTEAEIRKVMNGDYQTSYIEVKRGSKIGEKSTWMLNLSIDVPKIDKGVDPSIIGGIDVGVKSPLVCAINDALSRYSISDNDLFHFNKKMFARRRILLKKNSHKRAGHGAKNKLKPITILTEKSKRFRKKLIERWACEIADFFVKNKVGTVQMENLESMKRREDSYFNIRLRGFWPYAEMQDKIEFKLKQYGIEIRKVAPNNTSKTCSRCGHLNNYFNFEYRRKNKFPHFKCEKCNFKEDADYNAALNISNPKLKSTKGEP

SEQ ID NO: 2740 - protein, 726 aa, synthetic construct
SEVEFSHEYWMRHALTLARRARDEREVPVGAILVLNNRVIGEGWNRAIGLHDPTAHAEIMALRQGGLVMQNYRLTDATLYVTFEPCVMCAGAMIHSRIGRVVFGIRNSKRGAAGSQMNVLNYPGMNHRVEITEGILANECAALLCDFYRMPRQVFNARKKAQSSINPGGSSGGSSGSETPGTSESATPESSGGSSGSSAKNTITKALKLRIVRPYNSAEVEKIVADEKNNREKIALEKNKDKVKEACSKHLKVASYCTTQVERNACLFCKARRLDDKFYQKLRGQFPDAVFWQELGEIFRQLQKQAAEIYNQSLIELYYEIFIKGKGLANASSVEHYLSDVCYTRAAELFKNAAIASGLRGKVKSNFKLKELKSMKSGLPSTKSDNFPIPLVKQKGGQYTGFEISSHNDDLIIKIPFGRWQVKREIDKYRPWEKFDFEQVRKSPKPISLLLSTQRRKRNRGWSKDEGTEAEIRKVMNGDYQTSYIEVKRGSKIGEKSAWMLNLSIDVPKIDKGVDPSIIGGIDVGVKSPLVCAINNAFSRYSISDNDLFRFNKKMFARRRILLGKNRHKRAGHGVKNKLKPITILTEKSGRFRKKLIERWACEIADFFIKNKVGTVQMENLESMKRKEDSYFNIRLRGFWPYAEMQNKIELKLKQYGVKIRKVAPNNTSKTCSKCGHLNNYFNFEYRKKNKFPHFKCEKCNFKEDADYNAALNISNPKLRSTKEEP

SEQ ID NO: 2741 - protein, 726 aa, synthetic construct
SEVEFSHEYWMRHALTLAKRARDEREVPVGAVLVLNNRVIGGGWNRAIGLHDPTAHAEIMALRQGGLVMQNCRLVDATLYVTFEPCVMCAGAMIHSRIGRVVFGVRNSKRGAAGSLMNVLNYPGMNHRVEITEGILAGECAALLCDFYRMPRQVFNAQKKAQSTINSGGSSGGCSGSEMPGASESVTPKSSGGSSAGSTKNTITKTLKLRIVRPYNSAEVEKIVADEKNSREKIALERNKDKVKEACSEHLKVAAYCTTQVERNACLFCKARKLDDKFYQKLRGQFPDAVFWQEIGEIFRQLQKQAAEIYNQSLIELYYEIFIKGKGFANTSSVEHYLSDVCYTRAAELFKNAAIASGLRGKVKSNFRLKELKNMRSGLPTAKSDNFPIPLVKQKGGQYTGFEISSHNDDFIVKIPFGRWQVKKEIDKYRPWEKFDFEQVRKSPKPISLLLSTRRRKRNKGWSKDEGTEAEIKKVMNGDYQTSYIEVKRGSKVGEKSAWMLNLSIDVPKIDKGVDPSIIGGIDVGVKSPLVCAINNAFSRYSISDNDLYRFNKKMFARRRILLKKSKHKRAGHGAKNKLKPITILTEKSGRFRKKLIERWACEIADFFVKNKVGTVQMENLESMKRREDSYFNIRLRGFWPYAEMQNKIEFKLKQYGIEIRKVAPNNTSKTCSKCGHLNSYFNFEYRKKNKFPHFKCEKCNFKENADYNAALNISNPKLKSTKEVP

SEQ ID NO: 2742 - protein, 726 aa, synthetic construct
SEVEFSHEYWMRHALTLAKRARDGREVPVGAVLVLNNRVIGEGWNRAIGLHDPTAHAEIMALRQGGLVMQNYRLIDATLYVTFEPCVMCAGAMIHSRIGRVVFGVRNSKHGAAGSLVNVLNYPGMNHRVEITEGILADECAALLCDFYRMPRQVFNARKKAQSSINPSGSSGGSSGSVTPGTSESATPESSGGGFGGSAKNTITKTLQLRIVRPYNSAEVEKIVADEKNNREKIALEKNKDKVKEACSEHLKVAAYCTTQVERNACLFCKARKLDDKFYQKLRGQFPDAVSWQEIGEIFRQLQKQAAEIYNQSLIELYYEIFIKGKGFANASSVEHYLSDVCYTRAAELFKNAAIASGLRGKVKSNFRLKELKNMKSGLPTTKSDNFPIPLVKQKGGQYTGFEISSHNDDFIIKIPFGRWQVKKEINKHRPWEKFDFERVRKSPKPISLLLSTQRRKRNKGWSKDEGTEAEIRKVMNGDYQTSYIEVKRGSKIGEKSAWMLNLSIDVPKIDKGVDPSIIGGIDVGVKSPLVCAINNALSRYSISDNDLFHFNKKMFARRRILLRKNGHKRAGHGAKNKLKPITIMTEKSKRFRKKLIERWACEIADFFVKNKVGTVQMENLESMKRKEDSYFNVRLRGFWPYAEMQNKIEFKLKQYGIKIRKVAPNNTSRTCSKCGHLNSYFSFEYRKKNKFPHFKCEKCNFKEDADYNAALNISNPRLKSTKEEP

SEQ ID NO: 2743 - protein, 726 aa, synthetic construct
SEVEFSHEYWMRHALTLAKRARDEREVPVGAILVLNNRVIGEGWNRAIGLHDPTAHAEIMALRQGGLVMQNHRLVDATLYVTFEPCVMCAGAMIHSRIGRVVFGVRNSKRGAAGSLTNVLDHPGMNHRVEITEGILGDECAALLCDFYRMPRQVFNAQKKAQSTINSGGSSGGSSGSETPCTSESATPKSSGGSSGGSAKNTITKTLKLRIVRPYNSAEVEKIVADEKDSREKIALEKNKDKVKEACSKHLKVAAYCTTQVERNACLFCKARKLDDKFYQKLRGQFPDAVFWQELGEILRQLQKQVAEIYNQSLIELYYEIFIKGKGIANASSVEHYLSDVCYTRAAELFKNAAIASGLRSKVRSNFRLKELKSMKSGLPTTKSDNFPIPLVKQKGGQYTGFEISSHNGDFIIKIPFGRWQVKEEIDRFRPWEKFDFEQVRKSPKPISLLLSTQRRKKNKGWSKDEGTEAEIRKVMNGDYQTSYIEVKRGSKVGEKSAWMLNLSIDVPKIDRGVNPSIIGGVDVGVKSPLVCAINNALSRYSVSDNDLFRFNKKMFARRRILLKKNRHKRAGHGAKNKLKPITILTKKSERFRKKLIERWACEIADFFIKNKVGTVQMENLESMKRREDSYFNIRLRGFWPYAEMQNRIEFKLKQFGIEIRKVAPHNTSKTCSKCGHLNNYFNFEYRKKNKFPHFKCEKCNFKEDADYNAALNISNPKLKSTKEEP

SEQ ID NO: 2744 - protein, 726 aa, synthetic construct
SEVEFSHEYWMRRALTLAKRARDEREVPVGAVLVLNNRVIGVGWNRAVGLHDPTAHAEIMALRQGGLVMQNYRLIEATLYVTFEPCIMCAGAMIHSRIGRVVFGVRNSKRGAAGSLVNVLNYPGMNHRVEITEGILVDECAALLCDFYRMPRQVLSAQKRAQSSISSGGSSGGSSGSETPGTSGGVTPKSSVGSSAGSTKNTITKTLKLRIVRPYNSAEVEKIVADEKNNREKIALEKNKDKVKEACSKHLKVAAYCTTQVERNACLFCKARKLDDKFYQKLRGQFPDAVFWQEIGEIFRQLQKQAAEIYNQSLIELYYEIFIKGKGFANASSVEHYLSDVCYTRAAELFKNAAIASGLRGKVKSNFRLKELKNMKSGLPTTKSDNFPIPLVKQKGGQYTGFEISSHNDDFIIKIPFGRWQVKKEINKYRPWEKFDFEQVRKSPKPISLLLSTRRRKRNKGWSKDEGTEAEIRKVMNGDYQTSYIEVKRGSKTGEKSAWMLNLSIDVPKVDKGVDPSIIGGIDVGVKSPLVCAINNAFSRYSISDNDLFRFNKKMFARRRILLGKNRHKRAGHGAKNKLKPISILTEKSERFRKKLIERWACEIADFFIKNKVGTVQMENLESMKRREDSYFNTRLRGFWPYAEMQNKIEFKLKQYGIEIRKVAPNNTSKTCSKCGHLNNYFNFKYRKKNKFPHFKCEKCNFKENADYNAALNISNPRLKSTKEEP

SEQ ID NO: 2745 - protein, 726 aa, synthetic construct
SEVEFSHEYWMRHALTLAKRARDEREVPVGAVLVLNNRVIGVGWNRAIGLHDPTAHAEIMALRQGGLVMQNYRLIDATLYVTFEPCIMCAGAMIHSRIGRVVFGVRNSKRGAAGSLMNVLNYPGMNHRVEITEGVLADECAALLCDFYRMPRQVLNAQKKAQSSINSGGSSGGSSGSETPGASESATPKSSGGSSAGSTKNTITKTLKLRIVRPYNSAEVEKIVADEKDNRERIALEKNKDKVKEACSKHLKVAAYCATQVERNACLFCKARKLDDKFYQKLRGQFPDAVFWQEIGEIFRQLQKQAAEIYNQSLIELYYEIFIKGKGFANASSVEHYLSDVCYTRAAELFKNAAIASGLRGKVKSNFRLKELKNMKSGLPTTKSDNFPIPLVKQKGGQYTGFEISNHNSNFIIKIPFGRWQVKKEIDKYRPWEKFDFEQVRKSPKPISLLLSTRRRKRNKGWSKDEGTEAEIRKVMNGDYQTSYIEVKRGSKIGEKSAWMLNLSIDVPKIDKGVDPSIIGGIDVGVKSPLVCAINNALSRYSISDNELFHFNKKMFARRRILLKKNRHKRAGHGAKNKLKPISILTEKSERFRKKLIEKWACEIADFFIKNKVGTVQMENLESIKRKEDSYFNIRLRGFWPYAEMQNKIEFKLKQYGIEIRKVAPNNTSKTCSKCGHLNNYFNFEYRKKNKFPHFKCEKCNFKENADYNAALNISNPKLKSTKEEP

SEQ ID NO: 2746 - protein, 726 aa, synthetic construct
SEVEFSHEYWMRHALTLAKRARDEREVPVGAVLVLNNRVIGVGWNRAIGLHDPTAHAEIMALRQGGLVMQNYRLIDATLYVTFEPCIMCAGAMIHSRISRVVFGVRNSKRGAAGSLMNVLNYPGMNHRVEITEGVLADECAALLCDFYRMPRQVFNAQKKAQSNINPGGSSGSSRGSETPGTSESAAPGSSGGGSSGSAKNTITKTLKLRIVRPYNSAEVEKIVADEKNNREKIALEKNKDKVKEACSEHLKVAAYCTTQVERNACLFCKARKLDDKFYQKLRGQFPDAVFWQELGEILRQLQKQAAEIYNQSLIELYYEIFIKGRGFANASSVEHYLSDVCYTRAAELFKNAAIASGLRGKVKSNFRLKELKNMKSGLPTTKSDNFPIPLVKQKGGQYTGFEISDHNSDFIIKIPFGRWQAKKEIDKYRPWEKFDFEQVRKSPKPISLLLSTQRRKKNRGWSKDEGTEAEIKKVMNGDYQTSYIEVKRGSKIGEKSAWMLNLSIDVPKIDKGVDPSIIGGIDVGVKSPLVCAISNAFSRYSISDNDLFHFNKKMFARRRILLKKNRHKRAGHGAKNKLKPFTILTEKSGRFRKKLIERWVCEIADFFVKNKVGTVQMENLESMKRKEDSYFNIRLRGFWPYAEMQNRIEFKLKQYGIKVRKVAPNNTSKTCSKCGHLNSYFSFEYRKKNKFPHFKCEKCNFKENADYNAALNISNPKLKSTKEEP

SEQ ID NO: 2747 - protein, 726 aa, synthetic construct
SEVEFSHEYWMRHALTLAKRARDEREVPVGAVLVLNNRVIGEGWNRAIGLHDPTAHAEIMALRQGGLVLQNYRLVDATLYVTFEPCVLCAGAMVHSRIGRVVFGARNSKRGAAGSLMNILNYPGMNHRVEITEGILADECAALLCDFYRMPRQVFNAQKKAQSSINSGGSSGGSSGSETLGTREGATPESTGGSSAGSTKDTITKTLKLRIVRPYNSAEVEKVVADEKNNREKIAMEKNKDKVKEACSKHLKVASYCTTQVERNACLFCKARKLDDKFYQKLRGQFPDAVFWQELGGIFRQLQKQAAEIYNQSLIELYYEIFIKGKGLANASSVEHYLSDVCYTRAAELFKNAAIASGLRGKVKSNFKLKELKSMKSGLPSTKSDNFPIPLVKQRGGQYTGFEISSHNDDFIIKIPFGRWQAKKEIDKYRPWERFDFEQVRKSPKPISLLLSTQRRKRNKGWSKDEGTEAEIRKVMNGDYQTSYIEVKRGSKTGEKSAWMLNLSIDVPKIDKGVDPSIIGGIDVGVRSPLVCAINNSFSRYSICDNDLFRFNKKMFARRRILLKKSRHKRAGHGAKNKLKPISILTEKSKRFRKKLIERWACEIADFFIKNKVGTVQMENLESMKRKEDSYFNIRLRGFWPYAEMQNKIEFKLRQYGIVVRKVAPNNTSKTCSQCGHLNNYFNFEYRKKNKFPHFKCEKCNFKENADYNAALNISNPKLKSPKEEP

SEQ ID NO: 2748 - protein, 726 aa, synthetic construct
SEVEFSHEYWMRHALTLAKRARDEREVPVGAVLVLNNRVIGEGWNRAIGLHDPTAHAEIMALRQGGLVMQNYRLTDATLYVTFEPCVMCAGAMIHSRIGRVVFGVRNSKRGAAGSLMNVLNYPGVNHCVEITEGILVDECAALLCDFYRMPRRVLNAQKKAQSSISSGGPSGGCSGSEMPGASESVTPKSSGGSSGGSTKNTITKTLKLRIVRPYNSAEVEKIVADEKNNREKIALEKNKGKVKEACSKHLKVATYCTTQVERNACLFCKARKLDDKFYQKLRGQFPDAVFWQEVGEIFRQLQKQAAEIYNQSLIELYYEIFIKGKGIANASSVGHYLSDVCYTRAAELFKNAAIASGLRGKVKSNFRPKELKNMKSGLPTTKSDNFPIPLVKQKGGQYTGFEISSHNDDLIIKIPFGRWQVKKEIDKYRPWEKFDFEQVRKSPKPISLLLSTQRRKRNKGWSKDEGTEAEIRKVMNGDYQTSYIEVKRGSKIGEKSAWMLNLSIDVPKIDKGVDPSIIGGIDVGVKSPLVCAINNAFSRYSISDNDLFHFNKKMFARRRILLKKNGHKRAGHGAKNKLRPITIMTEKSKRFRKKLIERWACEIADFFIKNKVGTVQMENLESMRRKEDSYFNIRLRGFWPYAEMQNKIEFKLKQYGIEIRKVAPNNTSKTCSKCGHLNNYFNFEYRRRNKFPHFKCEKCNFKEDADYNAALNISNPKLKGTKEEP

SEQ ID NO: 2749 - protein, 726 aa, synthetic construct
SEVEFSHEYWMRHALTLAKRARDEREVPVGAILVLNNRVIGEGWNRAIGLHDPTAHAEIMALRQGGLVMQNYRLIDATLYVTFEPCVMCAGAMIHSRIGRVVFGVRNSKHGAAGSLVNVLNYPGMNHRVEITEGILADECAALLSDFYCMPRQVFNAQKGAQSSINSGGSSSGSSGSDTPGTSESATPESSGGGSSGSAKNTITKTLQLRIVRPYNSAEVEKIVADEKNNREKIALEKNKDKVREACSKHLKVASYCTTQVERNACPFCKARKLDDRFYQKLRGQFPDAVFWQETGEIFRQLQRQAAEIYNQSLIELYYEIFIKGKGFANASSVEHYLSDVCYTRAAELFKNAAIASGLRGKVKSNFRLKELKNMKSGLPTTKSDNFPIPLVKQKGGQYTGFEISSHNDDFIIKIPFGRWQVKKEIDRYRPWEKFDFEQVRKSPKPISLLLSTQRRKRNKGWSKDEGTEAEIRKVMNGDYQTSYIEVKRGSKIGEKSAWMLSLSIDVPKIDKGVDPSTIGGIDVGVKSPLVCAINNAFCRYSISDNDLFHFNKKMFARRRILLKKSRHKRAGHGAKNKLKPISILTEKSKRFRKKLIERWACEIADFFIKNKVGTVQMENLESMKRKEDSYFNIRLRGFWPYAEMQNKIEFKLKQYGIKIRKVAPNNTSKTCSKCGHLNNYFNFEYRKKNKFPHFKCEKCNFKENADYNAALNISNPKLKSTKEEP

SEQ ID NO: 2750 - protein, 726 aa, synthetic construct
SEVEFSHEYWMRHALTLAKRARDEREVPVGAVLVLNNRVIGEGWNRAIGLHDPTAHAEIMALRQGGLVLQNYRLVDATLYVTFEPCVLCAGAMVHSRIGRVVFGARNSKRGAAGSLMNILNYPGMNHRVEVTEGILADECAALLCDFYRMPRQVFNAQKKAQSSINSGGSSGGSSGSETPSTSESATPESSSGSSGGSAKNTITKTLQLRIVRPYNSAEVEKIVTDEKNNREKIALEKNKDKVKEACSKHLKMASYCTTQVERNACLFCKARKLDDKFYQKLRGQFPDAVFWQELGGIFRQLQKQAAEIYNQSLIELYYEIFIKGKGITNASRVEHYLSDVCYTRAAELFKNAAIASGLRSKVRSNFRLKELKNMRSGLPTTKSDNFPIPLVKQKGGQYTGFEISSHNSDFIIKIPFGRWQVKEEIDKYRPWEKFDFEQVRKGPKPISLLLSTQRRKKNKGWSKDEGTEAEIRRVMNGDYQTSYIEVKRGSKIGEKSAWMLNLSIDVPKIDKGVDPSIIGGIDVGVKSPLVCAINNALGRFSISDNDLFHFNKKMFARRRILLRKNRHKRAGHGAKNKLKPISILTEKSRRFRKKLIERWACEIADFFIKNKVGTVQMEDLESMKRKEDSYFNIRLRGFWPYAEMQNKIEFKLKQYGIEIRKVAPNNTSKTCSKCGHLNNYFNFEYRKKNKFPHFKCEKCNFKENADYNAALNISNPKLKSTKEEP

SEQ ID NO: 2751 - protein, 726 aa, synthetic construct
SEVEFSHEYWMRHALTLAKRARDEREVPVGAILVLNNRVIGEGWNRAIGLHDPTAHAEIMALRQGGLVMQNYRLTDATLYVTFEPCVMCAGAMIHSRIGRVVFGVRNSKHGAAGSLVNVLNYPGMNHCVEITEGILVDECAALLCDFYRMPRQVLNAQKKAQSSISSGGSSGGSSGSETPGAGESVTPKSSVGSSAGSTKNTITKTLKLRIVRPYNSAEVEKIVADEKNNREKIALEKNKDKVKEACSKHLKVASYCTTQVERNACLFCKARKLDDKFYQKLRGQFPDAVFWQELGEIFRQLQKQAAEIYNQSLIELYYEIFIKGKGFANASSVEHYLSDVCYTRAAELFKNAAIASGLRGKVKSNFRLKELKNMKSGLPTTKSDNFPIPLVKQKGGQYTGFEISSHNDDFIIKIPFGRWQVKKEIDKYRPWEKFDFEQVRKSPKPISLLLSTQRRRRNKGWSKDEGTEAEIRKVMNGDYQASYIEVKRGSKIGEKSAWMLNLSIDVPKIDKGVDPSIIGGIDVGVKSPLVCAINNAFSRYSISDNDLFHFNKKVFARRRILLKKNRHRRAGHGAKNKLKPITILTEKSVRFRKKLIERWACEIADFFVKNKVGTVQMENLEGMKRKEDSYFNIRLRGFWPYAEMQNKIEFKLKQYGIEVRKVAPNNTSKTCSKCGHLNNYFNFEYRKKYKFPHFKCEKCNFKENADYNAALNISNPKLKSTKEEP

SEQ ID NO: 2752 - protein, 726 aa, synthetic construct
SEDEFSHEYWMRHALTLAKRARDGREVPVGAVLVLNNRVIGEGWNRAIGLHDPTAHAEIMALRQGGLVMQNYRLIDATLYVTFEPCVMCAGAMVHSRIGRVVFGVRNSKRGAAGSLMNVLDYPGMGHRVEITEGILADECAALLCDFYCMPRQVFNAQKRAQSSINSGGSSGGSSGSDTPGTSESATPESSGGSSGSSAKNTITKTLKLRIVRPYNSAEVEKIVADEKNNREKIALEKNKDKVKEACSQHLKVATYCTTQVERNACLFCRARKLDDEFYQKLRGQFPDAVFWQEISEIFRQLQKQAAEIYNQSLIELYYEIFIKGKGFANASSVEHYLSDVCYTRAAGLFKNAAIASGLRGKVKSNFRLKELRNMKSGLPTTKSDNFPIPLVRQKGGQYTGFEISNHNSDFIIKIPFGRWQAKREIDKYRPWEKFDFEQVRKSPKPISLLLSTQRRKRSRGWNKDEGTEAEIRKVMNGDYQTSYIEVKRGSKIGEKSAWMLNLSIDVPRVDKGVDPSIIGGIDVGVKSPLVCAINNAFSRYSISDNDLFRFNKKMFARRRILLGKNRHKRAGHGVKNKLKPISILTGKSERFRKKLIERWACEIADFFIKNKVGTVQMENLESMKRKEDSYFNIRLRGFWPYAEMQNKIEFKLKQYGIEIRKVAPNDTSKTCSKCGHLNNYFNFEYRKKNKFPHFKCEKCNFKENADYNAALNISNPKLKSTKEEP

SEQ ID NO: 2753 - protein, 726 aa, synthetic construct
SEVEFSHEYWMRHALTLAKRARDGREVPVGAVLVLNNRVIGEGWNRAIGLHDPTAHAEIMALRQGGLVMQNYRLINATLYVTFEPCVMCAGAMVHSRIGRVVFGVRNSKRGAAGSLMNVLDYPGMGHRVEITEGILADECAALLCDFYCMPRQVFNAQKRAQSSINSGGSAGGSSGSETPGTSESATPGSFGGGSSGSARNTITKTLQLRIVRPYNSAEVEKIVADEKNNREKIALEKNKDKVKEACSKHLKVASYCTTQVERNACPFCKARKLDDKFYQKLRGQFPDAVFWQELGEILRQLQKQAAEVYNQSLIELYYEIFIKGRGFANASSVEHYLSDVCYTRAAELFKNAAIASGLRGKVKSNFRLKELRNMKSGLPTTKSDNFPIPLVRQKGGQYTGFEISSHDGDFIIKIPFGRWQVKKEINKHRPWEKFDFEQVRKSPKPISLLLSTQRRKRNKGWSKDEGTEAEIRKVMNGDYQTSYIEVKRGSKIGEKSAWMLNLSIDVPKIDKGVDPSIIGGIDVGVKSPLVCAINNAFSRYSISDNDLFHFNKKMFARRRILLKKNRHRRAGHGARNKLKPITVLTEKSKRFRKKLIERWACEIANFFIKNKVGTVQMENLESMKRKEDSYFNIRLRGLWPYAEMQNKIEFKLKQYGIEIRKVAPNNTSKTCSKCGHLNNYFNFEYRKKNKFPHFKCEKCNFKENADYNAALNISNPKLKSTKEEP

SEQ ID NO: 2754 - protein, 726 aa, synthetic construct
SEVEFSHEYWMRHALTLAKRARDEREVPVGAILVLNNRVIGEGWNRAIGLHDPTAHAEIMALRQGGLVMQNYRLIDATLYVTFEPCVMCAGAMIHSRIGRVVFGVRNSKHGAAGSLVNVLNYPGMNHRVEITEGILADECAALLCDFYRMPRRVFNARMKAQSTINSGGSSGGSSSSETPGTSESASPEGSGGSSGGSAKNTITKTLKLRIVRPYNSAEVEKIVADEKNNREKIALEKNKDKVKEACSKHLKVASYCTTQVERNACLFCKARKLDDKFYQKLRGQFPDAVFWQELGEIFRQLQKQAAEIYNQSLIELYYQIFIKGKGFANASSVEHYLSDVCYTRAAELFKNAAIASGLRGKVKSNFRLKELKNMKSGLPTTKSGNFPIPLVKQKGGQYTGFEISSHNDDFIIKIPFGRWQMKKEVDKYRPWEKFDFEQVRKSPKPISLLLSTQRRKRNKGWSKDEGTEAEIRKVMNGDYQTSYIEVKRGSKIGEKSAWMLNLSIDVPKIDKGVDPSIIGGIDVGVRSPLVCAIDNAFSRYSISDNDLFHFNKKMFARRRILLKKNRHKRAGHGAKNKLKPISILTEKSKRFRKKLIERWACEIADFFIKNKVGTVQMENLESMKRKEDSYFNIRLRGLWPYAEMQDKIEFKLKQYGIEIRKVAPNNTSKTCSRCGHLNNYFNFEYRRRNKFPHFKCEKCNFKENADYNAALNISNPKLKSTKEEP

SEQ ID NO: 2755 - protein, 726 aa, synthetic construct
GGVEFSHEYWMRRALTLAKRARDEREVPVGAVLVLNNRVIGEGWNRAIGLHDPTAHAEIMALRQGGLVMQNYRLIGATLYVTFEPCAMCAGAMIHSRIGRVVFGVRNSKHGAAGSLVNVLNYPGMGHRVEITEGILVDECAALLCDFYRMPRQVLNAQKKAQSSISSGGSSGGSSCSETPGASESVTPKSSGGSSAGSTKNTITKTLKLRIVRPYNSAEVEKIVADEKNNREKIALEKNKDKVQEACSKHLKVASYCTTQVERNACLFCKARKLDDKFYQKLRGQFPDAVFWQELGEIFRQLQKQAAEIYNQSLIELYYEIFIKGKGFANASSVEHYLSDVCYTRAAELFKNAAIASGLRGKVKSNFRLRELKNMKSGLPTTKSDNFPIPLVKQKGGQYTGFEISNHNSDFIIKIPFGRWQVKKEINRYRPWEKFDFEQVRKSPKPISLLLSTQRRKRNKGWGKDEGTEAEIRKVMNGDYQTSYIEVKRGSKIGEKSAWMLNLSIDVPKIDKGVDPSIIGGVDVGVKSPLVCAINNAFSRYSIGDNDLFHYNKKMFARRRILLKKNRHKRAGHGAKNKLKPISILTEKSKRFRKKLIERWACEIADFFIRNKVGTVQIENLESMKRREDSYFNIRLRGFWPYAEMQNKIEFKLKQYGIEIRKVAPNNTSKTCSKCGHLNSYFNFEYRKKNKFPHFKCEKCNFKENADYNAALNISNPKLKSTKEEP

SEQ ID NO: 2756 - protein, 726 aa, synthetic construct
SEDEFSHEYWMRHALTLAKRARDGREVPVGAVLVLNNRVIGEGWNRAIGLHDPTAHAEIMALRQGGLVMQNYRLIDATLYVTFEPCVMCAGAMVHSRIGRVVFGVRNSKRGAAGSLMNVLDYPGMGHRVEITEGILADECAALLCDFYCMPRQVFNAQKRAQSSINSGGSSGGSSGSETPGTSESATPESSGGGSSGSAKSTITKTLQLRIVRPYNSAEVEKIVADEKNNREKIALEKNKDKVKEACSKHLKVASYCTTQVERNACPFCKARKLDDKFYQRLRGQFPDAVFWQELGEILRQLQKQAAEIYNQSLIELYYEIFIKGRGFANASSVEHYLSDVCYTRAAELFKNAAIASGLRGKVKSNFRLKELKNMKSGLPTTKSDNFPIPLVKQKGGQYTGFEISSHNDDFIIKIPFGRWQVKKEIDKYRPWEKFDFEQVRKSPKPISLLLSTQRRKRNKGWSKDEGTEAEIRKVMNGDYQTSYVEVKRGSKTGEKSAWMLNLSIDVPKIDKGVDPSIIGGIDVGVKSPLVCAINNAFSRYSISDNDLFRFNKKMFARRRILLKKNRHKRAGHGAKNKLKPISALTEKSGRFRKKLIERWACEIADFFIKNKVGTVQMENLGSMKRKEDSYFNIRLRGFWPYAEMQNKIEFKLKQYGIEIRKVAPDNTSKTCSKCGHLNNYFNFEYRKKNKFPLFKCEKCNFKENADYNAALNISNPKLKSTKGEP

SEQ ID NO: 2757 - protein, 726 aa, synthetic construct
SEVEYSHEYWMRHALTLAKRARDEREVPVGAILVLNNRVIGVGWNRAIGLHDPTAHAEIMALRQGGLVMQNYRLIDATLYVTFEPCVMCAGAMIHSRIGRVVFGVRNSKHGAAGSLVNVLNYPGMNHRVEITEGILVDECAALLCDFYCMPRQVLNAQKKAQSSISPGGSSGGGSGSETPSTSENTTPESSGGSSGGPAKNTITKTLKLRIVRPYNSAEVEKIVADEKNNREKTALERNKDKVKEACSKHLKMAAYCTTQVERNACLFCKARKLDDKFYQKLRGQFPDAVFWQEVGEIFRQLQKQAAEIYNQSLIELYYEIFIKGKGFANASSVEHYLSDVCYTRAAELFKNAAIASGLRGKVKSNFRLKELKNMKSGLPTTKSDNFPIPLVKQKGGQYTGFEISSHNDDFIIKIPFGRWQVKEEVDKYRPWEKFDFEQVRKNPKPISLLLSTQRRKRNRGWSKDEGTEAEIRKVMNGDYQTSYIEVKRGSKIGEKSAWTLSLSIDVPKIDKGVDPSIIGGIDVGVKSPLVCAINNALSRYSISDNDLFHFNKKMFARRRILLRKNRHKRAGHGARNKLKPITVLTGKSERFRKKLIERWACEIADFFIKNKVGTVQMENLESMKRKEDSYFNIRLRGFWPYAEMQNKIEFKLKQYGIEIRKVAPNNTSKTCSKCGHLNNYFNFEYRKKNKFPHFKCEKCNFKEDADYNAALNISNPKLKSTRGEP

SEQ ID NO: 2758 - protein, 726 aa, synthetic construct
SEVEFSHEYWMRHALTLAKRARDEREVPVGAVLVLNNRVIGEGWNRAIGLHDPTAHAEIMALRQGGLVMQNYRLIDATLYVTFEPCVMCAGAMIHSRIGRVVFGVRNSKRGAAGSLMNVLDYPGMNHRVEITEGILTDECAALLCDFYRMPHQVLNAQRKAQSNINSGGSSGGSSGSETPGTSESPTPESSGGSSGGSAKNTITKTLKLRIVRPYNSAEVEKIVADEKNNREKIALEKNKDKVREACSKHLKVAAYCTTQVERNACLFCRARKLDDKFYQKLRGQFPDAVFWQEIGGIFRQLQKQAAEIYNQSLIELYYEIFIKGKGFANTSSVEHYLSDVCYTRAAELFKNAAIASGLRGKVKSNFRLKELKNMKSGLPTTKSDNFPIPLVKQKGGQYTGFEISSHNDDFIIKIPFGRWQVKKEIDKYRPWEKFDFEQVRKSPKPISLLLSTQRRKRNKGWSKDEGTEAEIRKAMNGDYQTSYIEVKRGSKIGEKSAWMLNLSIDVPKIDKGVDPSIIGGIDVGVKSPLVCAINNAFSRYSISDNDLFRFNKKVFARRRILLKKNRHKRAGHGTKNKLKPITILTEKSGRFRKKLIERWACEIANFFIKNKVGTVQMENLESMKRREDSYFNIRLRGFWPYAEMQNKIEFKLKQYGIEIRKVAPNNTSKTCSKCGHLNNYFNFEYRKKSKFPHFKCEKCNFKENADYNAALNISNPKLKGTKEEP

SEQ ID NO: 2759 - protein, 726 aa, synthetic construct
SEVEFSHEYWMRHALTLAKRARDEREVPVGAILVLNNRVIGEGWNRAIGLHDPTAHAEIMALRQGGLVMQNYRLIDATLYVTFEPCVMCAGAMIHSRIGRVVFGVRNSKRGAAGSLMNVLNYPGVNHRVEITEGILVDECAALLCDFYRMPRQVLNAQKKAQSSISSGGSSGGCSGSEMPGASESVTPKSSGGSSAGSTKNTITKTLKLRIVRPYNSAEVEKIVADEKNNREKIALEKNKDKVKEACSKHLKVAAYCTTQVERNACLFCKARRLDDKFYQKLRGQFPDAVFWQEIGEIFRQLQRQAAEIYNRSLIELYYEIFIKGKGFANASSAEHYLSDVCYTRAAELFKNAAIASGLRGKVKSNFRLKELKNMKSGLPTTKSDNFPIPLVKQKGGQYTGFEISSYNDDFIIKIPFGRWQVKKEIDRYRPWEKFDFEQVRKSPKPISLLLSTQRRKRNKGWSKDEGTEAEIRKVMNGDYQTSYIEVKRGSKIGEKSAWMLNLSIDVPKIDKGVDPSIIGGIDVGVKSPLVCAINNALSRYSISDNDLFHFNKKMFARRRILLRKNRHKRAGHGAKNKLKPITMMTEKSKRFRKKLIERWACEIADFFIKNKVGTVQMENLESMKRKEDSYFNIRLRGFWPYAEMQDKIEFKLKQYGIVVRKVAPNNTSKTCSKCGHLNHYFSFEYRKKNKFPHFKCEKCNFKEDADYNAALNISNPKLKSTKGEP

SEQ ID NO: 2760 - protein, 726 aa, synthetic construct
SEVEFSHEYWMRHALTLAKRARDEREVPVGAVLVLNNRVIGEGWNRTTGLHDPTAHAEIMALRQGGLVMQNHRLVDATLYVTFEPCVMCAGAMIHSRIGRVVFGVRNSKRGAAGSLTNVLNYPGMNHRVEITEGILVDECAALLCDFYRMPRQVFNAQKKAQSNINSGGSSGGSSGSETPGTSESPTPESSGGSSGGSAKNTITKTLKLRIVRPYNSAEVEKIVADEKNNREKIALEKNKDKVREACSKHLKVAAYCTTQVERNACLFCRARKLDDKFYQKLRGQFPDAVFWQEIGGIFRQLQKQAAEIYNQSLIELYYEIFIKGKGFANTSSVEHYLSDVCYTRAAELFKNAAIASGLRGKVKSNFRLKELKNMKSGLPTTKSDNFPIPLVKQKGGQYTGFEISSHNDDFIIKIPFGRWQVKKEIDKYRPWEKFDFEQVRKSPKPISLLLSTQRRKRNKGWSKDEGTEAEIRKAMNGDYQTSYIEVKRGSKIGEKSAWMLNLSIDVPKIDKGVDPSIIGGIDVGVKSPLVCAINNAFSRYSISDNDLFHFNKKMFARRRILLKKNRHRRAGHGAKNKLKPIAVLAEKSEGFRKKLIERWACEVADFFIKNKVGTVQMENLESMKRREDSYFNIRLRGFWPYAEMQNKIEFKLRQYGIEIRKVAPNNTSKTCSKCGHLNNYFDFEYRKKNKFPHFKCEKCNFKEDADYNAALNISNPKLKSTKEEP

SEQ ID NO: 2761 - protein, 726 aa, synthetic construct
SEVEFSHEYWMRHALTLAKRARDEREVPVGAILVLNNRVIGEGWNRAIGLHDPTAHAEIMALRQGGLVMQNYRLIDATLYVTFEPCVMCAGAMIHSRIGRVVFGVRNSKHGAAGSLVNVLNYPGMNHRVEITGGILADECAALLCDFYRMPRQVFNARKKARSSINPGGSSGGSSGSETPGTSKSATPESSGGSSGGPAKNTITKTLQLRIVRPYNSAEVEKIVADEKNNREKIALEKNKDKVKEACSEHLKVAAYCTTQVERNACLFCKARKLDDKFYQKLRGQFPDAVFWQELGEILRQLQKQAAEIYNQSLIELYYEIFIKGRGFANASSVEHYLSDVCYTRAAELFKNAAIASGLRGKVKSNFRLKELKNMKSGLPTTKSDNFPIPLVKQKGGQYTGFEISSHNDDIIIKIPFGRWQVKKEIDKYRPWEKFDFEQVRKSPKPISLLLSTQRRKRNKGWSKDEGTEAEIRKVMNGDYQTSYIEVKRGSKTGEKSAWMLNLSIDVPKIDKGVDPSIIGGIDVGVKSPLVCAINNALSRYSISDNDLFHFNKKMFARRRILLKKTRHKRAGHGAKNKLKPITVLTEKSERFRKKLIERWACEIADFFIKNKVGIVQMENLESMKRREDSYFNIRLRGFWPYAKMLNKIEFKLKQYGIEIRKVAPNNTSKTCSKCGHLNSYFNFEYRKKNKFPPFKCEKCNFKEDADYNAALNISNPKLKSTKEEP

SEQ ID NO: 2762 - protein, 726 aa, synthetic construct
SEVEFSHEYWMRHALTLAKRARDEREVPVGAILVLNNRVIGEGWNRAIGLHDPTAHAEIMALRQGGLVMQNYRLTDATLYVTFEPCVMCAGAMIHSRIGRVVFGVRNSKRGAAGSLMNVLNYPGMNHCVEITEGILVDECAELLCDFYRMPRQVLNARKKAQSSISSGGSSGGSSGSETPGASESATPKSSGGSSASSTKNTITKTLKLRIVRPYNSAEVEKIVADEKNNREKTALEKNKDKVKEACREHLKVAAYCTTQVERSACLFCKARKLDDRFYQKLRGQFPDAVFWQEISEIFRQLQKQAAEIYNQSLIELYYEVLIKGKGIANASSVGHYLSDVCYTRAAELFKNAAIASGLRSKIKSNFRLKELRNMRGGLPTTKSDNFPIPLVKQKGGQYTGFEISSHNDDFIIKIPFGRWQVKKEIDKYRPWEKFDFEQVRKSPKPISLLLSTQRRKRNKGWSRDEGTEAEIRKVMNGDYQTSYIEVKRGSKTGEKSAWMLNLSIDVPKINKGVDPSIIGGIDVGVKSPLVCAINNAFSRYSISDNDLFRFNKKMFARRRILLKKNRHKRAGHGAKNKLKPISILTGKSERFRKKLIERWACEIADFFIKNKVGTVQMENLESMKRKEDSYFNIRLRGFWPYAEMQNKIEFKLKQYGIEIRKVAPNNTSKTCSKCGHLNNYFNFEYRKKNKFPHFKCEKCNFKENADYNAALNISNPKLKSTKEEP

SEQ ID NO: 2763 - protein, 726 aa, synthetic construct
SEVEFSHEYWMRHALTLAKRARDAREVPVGAILVLNNRVIGEGWNRAIGQHDPTAHAEIMALRQGGLVMQNYRLTDATLYVTFEPCVMCAGAMIHSRIGRVVFGVRNSKRGAAGSLMNVLNYPGMNHCVEITEGILVDECAALLCDFYRMPRQVLNAQKKAQSTINSGGSSGGSSGSETPGTSESATPKSSGGSSGGSAKNTITKALKLRIVRPYNSAEVEKIVADEKNNRERIALEKNKDKVKEACSKHLKVAAYCTTQVERNACLFCKARKLDDKFYQKLRGQFPDAVFWQELGGIFRQLQKQAAEIYNQSLIELYYEIFIKGKGITNASRVEHYLSDVCYTRAAELFKNAAIASGLRGKVKSNFRLKELKNMKSGLPTTKSDNFPIPLVKQKGGQYTGFEISSHNDDFIIKIPFGRWQVKREIDKYRPWEKFDFEQVRKSPRPISLLLSTQRRKRNKGWSKDEGTEAEIRKVMNGDYQTSYIEVKRGSKIGEKSAWMLNLSIDVPKIDKGVDPSIIGGIDVGVKSPLVCAINNAFSRYSISDNDLFHFNKKMFARRRILLKKTRHKRAGHGAKNKLKPISILTEKSERFRKKLIERWACEIADFFIKNKVGTVQMENLESMKRREDSYFSTRLRGFWPYAKMQNKIEFKLKQYGIEIRKVAPNNTSKTCSKCGHLNNYFNFEYRKKNKFPHFKCEKCNFKENADYNAALNISNPKLKSTKEEP

SEQ ID NO: 2764 - protein, 726 aa, synthetic construct
SEVEFSHEYWMRHALTLAKRARDEREVPVGAVLVLNNRVIGEGWNRAIGLHDPTAHAEIMALRQGGLVMQNYRLVDATLYVTFEPCVMCAGAMIHSRIGRVVFGVRNSKRGAAGSLMNVLNYPGMGHRVEITEGILADECAALLCDFYCMPRQVFNAQKRAQSSINSGGSSGGSSGSETPGTSEGATPGSSGGGSSGSAKNTITKTLQLRIVRPYNSAEVEKIVADEKNNREKIALEKNKDKVKEACSKHLKVASYCTTQVERNACPFCKARKLDDKFYQKLRGQFPDAVFWQEIGEIFRQLQKQAAEIYNQSLIELYYEIFIKGKGFANAGSVEHYLSDVCYTRAAELFKNAAIASGLRNKIKSNFRLKELRNMKSGLPTTKSDNFPIPLVRQKGGRYTGFEISSHNDDFIIKIPFGRWQVKKEIDKYRPWEKFDFEQVRKSPKPISLLLSTRRRKRNKGWSKDEGTEAEIRKVMNGDYQTSYIEVKRGSKIGEKSAWMLSLSIDVPKIDKGVDPSIIGGIDVGVKSPLVCAINNAFSRYSISDNDLFHFNKRMFARRRILLRENGHKRAGHGAKNKLKPITIMTEKSKRFRKKLIERWACEIADFFIKNKVGTVQMENLESMKRREDSYFNIRLRGFWPYAEMQNKIEFKLKQYGIVVRKVAPNNTSKTCSKCGHLNNYFNFEYRKKNKFPHFKCEKCNFKEDADYNAALNISNPKLKSTKGEP

SEQ ID NO: 2765 - protein, 726 aa, synthetic construct
SEDEFSHEYWMRHALTLAKRARDGREVPVGAVLVLNNRVIGEGWNRAIGLHDPTAHAEIMALRQGGLVMQNYRLIDATLYVTFEPCVMCAGAMVHSRIGRVVFGVRNSKRGAAGSLMSVLDYPGMGHRVEITEGILADECAALLCDFYCMPRQVFNAQKRAQSSINSGGSSGGSSGSETPGTSESATPESSGGGSSGSAKSTITKTLQLRIVRPYNSAEVEKIVADEKNNREKIALEKNKDKVKEACSKHLKVASYCTTQVERNACPFCKARKLDDKFYQKLRGQFPDAVFWQELGEILRQLQKQAAEIYNQSLIELYYEIFIKGRGFANASSVEHYLSDVCYTRAAELFKNAAIASGLRGKVKSNFRLKELKNMKSGLPTTKSDNFPIPLVKQKGGQYTGFEISSHNDDFIIKIPFGRWQVKKEIDKYRPWEKFDFEQVRKSPKPISLLLSTQRRKRNKGWSKDEGTEAEIRKVMNGDYQTSYIEVKRGSKIGEKSAWMLNLSIDVPKVDKGVDPNIIGGIDVGVKSPLVCAINNALSRYSISDNDLFHFNKKMFARRRILLRKNRYKRAGHGARNKLKPITVLTEKSERFRKKLIERWACEIANFFIKNKVGTVQMEDLESMKRREDSYFNIRLRGFWPYAEMQNKIEFKLKQYGIEIRKVAPNNTSKTCSKCGHLNNYFNFEYRKMNKFPHFKCEKCNFKENADYNAALNISNPKLKGTKEEP

SEQ ID NO: 2766 - protein, 726 aa, synthetic construct
SEDEFSHEYWMRHALTLAKRARDGREVPVGAVLVLNNRVIGEGWNRAIGLHDPTAHAEIMALRQGGLVMQNYRLIDATLYVTFEPCVMCAGAMVHSRIGRVVFGVRNSKRGAAGSLMNVLDYPGMGHRVEITEGILADECAALLCDFYCMPRQVFNAQKRAQSSINSGGSSGGSSGSDTPGTSESATPESSGGGSSGSAKNTITKTLQLRIVRPYNSAEVEKIVADEKNSREKIALEKNKDKVKEACSKHLRVAAYCTTQVERNACLFCKARKLDDKFYQKLRGQFPDAVFWQEISEIFRQLQKQAAEIYNQSLIELYYEIFIKGKGIASASRVGHYLSDVCYTRAAELFKNAAIASGLRSKIKSNFRLKELKNMKSGLPTTKSDNFPIPLVKQKGGQYTGFEISNHNSDFIIKIPFGRWQVKKEIDKYRPWEKFDFEQVRKSPKPISLLLSTQRRRRNKGWGKDEGTEAEIRKVMNGDYQTSYIEVKRGSKIGEKSAWMLNLSIDVPKIDKGVDPSIIGGIDVGVKSPLVCAINNALSRYSISDNDLFHFNKKMFARRRILLRKNRHKRAGHGARNKLKPITVLTEKSERFRKKLIERWACEIANFFIKNKVGTVQMENLESMKRREDSYFNIRLRGFWPYAEMQSKIEFKLKQYGIKIRKVAPNNTSKTCSKCGHLNNYFNFEFRKKNKFPHFKCEKCNFKEDADYNAALNISNPKLKSTKEEP

SEQ ID NO: 2767 - protein, 726 aa, synthetic construct
SEVEFSHEYWMRHALTLAKRARDEHEVPVGAVLVLNNRAIGEGWNRAIGLHDPTAHAEIMALRQGGLVMQNYRLTDATLYVTFEPCVMCAGAMIHSRIGRVVFGVRNSKRGAAGSLMNVLNYPGMNHCVEITEGILVDECAALLCDFYRMPRQVLNAQKKAQSSISSGGSSGGSSGSETPGASGSVIPRSSGGSSAGSTKNTITKTLKLRIVRPYNSAEVEKIVADEKNNREKIALEKNKDKVKEACSKHLKVATYCTTQVERNACLFCKARKLDDKFYQKLRGQFPDAVFWQEVGEIFRQLQRQAAEIYNQSLIELYYEIFIKGRGFANASSVEHYLSDVCYTRAAELFKNAAIASGLRSKIKSNFRLKELRNMRGGLPTTKSDNFPIPLVKQKGGQYTGFEISSHNSDFVIKIPFGRWQVKEEIDKYRPWEKFDFEQVRKSPKPISLLLSTQRRKKNKGWSKDEGTEAEIRRVMNGDYQTSYIEVKRGSKIGEKSAWMLNLSIDVPKIDKGVDPSIIGGIDVGVKSPLVCAINNSFSRYSICDNDLFRFNKKMFARRRILLKKNRHKRAGHGAKNKLKPITILTKKSERFRKKLIERWVCEVADFFIKNKVGTVQMENLESMKRKEDSYFNIRLRGFWPYAEMQNRIELKLKQYGIEIRRVAPNNTSRTCSKCGHLNNYFNFEYRKKNKFPHFKCEKCNFKEDADYNAALNISNPKLKSTKEEP

SEQ ID NO: 2768 - protein, 726 aa, synthetic construct
SEVEFSHEYWMRHALTLAKRARDEREVPVGAVLVLNNRVIGEGWNRAIGLHDPTAHAEIMALRQGGLVMQNYRLIDATLYVTFEPCVMCAGAMVHSRIGRVVFGVRNSKRGAAGSLMNVLDYPGMGHRVEITEGILADECAALLCDFYCMPRQVFNAQKRAQSSINSGGSSGGSSGSDTPGTSESATPESSGGGSSGSAKNTITKTLQLRIVRPYNSAEVEKIVADEKNNREKIALEKNKDKVREACSKHLKVASYCTTQVERNACPFCKARKLDDKFYQKLRGQFPDAVFWQELGEILRQLQKQAAEIYNQSLIELYYEIFIKGKGLANASSVEHYLSDVCYTRAAELFKNAAIASGLRGKVKSNFKLRELKSMKSGLPSTKSDNFPIPLVKQRGGQYTGFEISSHNDDFIIKIPFGRWQAKKEIDKYRPWEKFDFEQVRKSPKPISLLLSTQRRKRNRGWSKDEGTEAEIRKVMNGDYQTSYIEVRRGSKIGEKNAWMLNLSIDVPKIDKGVDPSIIGGIDVGVKSPLVCAINNAFSRYSISDNDLFRFNKKMFARRRILLKKNRHKRAGHGAKNKLKPISILTGKSERFRKKLIERWACEIADFFIKNKVGTVQMENLESMKRKEDSYFNIRLRGFWPYAEMQNKIEFKLKQYGIEIRKVAPNNTSKTCSKCGHLNNYFNFEYRKKNKFPHFKCEKCNFKENADYNAALNISNPKLKSTREEP

SEQ ID NO: 2769 - protein, 726 aa, synthetic construct
SEVEFSHEYWMRHALTLAKRARDEREVPVGAILVLNNRVIGEGWNRAIGLHDPTAHAEIMALRQGGLVMQNYRLIDATLYVTFEPCVMCAGAMIHSRIGRVVFGVRNSKHGAAGSLVNVLNYPGMNHRVEITEGILADECAALLCDFYRMPRQVFNARKKTQSSINPSGSSGGSSGSVTPGTSESATPESSGGGFGGSAKNTITKTLQLRIVRPYNSAEVEKIVADEKNNREKIALEKNKDKVKEACSKHLKVASYCTTQVERNACLFCKARKLDDKFYQKLRGQFPDAVFWQELGEIFRQLQKQAAEIYNQSLIELYYEIFIKGKGFANASSVEHYLSDVCYARAAELFKNAAIASGLRGKVKSNFRLKELKNMKSGLPTTKSDNFPIPLVRQKGGQYTGFEISNHDGDFIIKIPFGRWQVKKEINKHRPWEKFDFEQVRKSPKPISLLLSTQRRKRNKSWSKDEGTEAEIRKVMNGDYQTSYIEVKRGSKIGEKSAWMLNLSIDVPKIDKGVDPGIIGGIDVGVKSPLVCAINNALSRYSISDNDLFHFNKKMFARRRILLRKNRHKRAGHGAKNKLKPITMMTEKSKRFRKKLIERWACEIADFFIKNKVGTVQMENLESMKRKEDSYFNIRLRGFWPYAEMQNKIEFKLKQYGIVVRKVAPNNTSKTCSKCGHLNNYFNFEYRKKNKFPHFKCEKCNFKEDADYNAALNISNPKLKSSKGEP

SEQ ID NO: 2770 - protein, 726 aa, synthetic construct
SEVEFSHEYWMRHALTLAKRARDEREVPVGAVLVLNNRVIGEGWNRAIGLHDPTAHAEIMALRQGGLVLQNYRLVDATLYVTFEPCVLCAGAMVHSRIGRVVFGARNSKRGAAGSLMNILNYPGMNHRVEITGGVLADECAALLCDFYRMPRQVFNAQKKAQSSINSGGSSGGSSGSETPSTSESPTPESSVGSSAGSTKNTITKTLKLRIVRPYNSAEVEKIVADEKNNREKIALEKNKDKVKEACSKHLKVAAYCTTQVERNACLFCKARKLDDMFYQKLRGQFPDAVFWQEIGEIFRQLQKQAAEIYNQSLIELYYEIFIKGRGFANASSVEHYLSDVCYTRAAELFKNAAIASGLRGKVKSNFRLKELKNMKSGLPTTKSDNFPIPLVKQKGGQYTGFEISSHNDDFIIKIPFGRWQAKKEIDKYRPWEKYDFEQVRKSPKPISLLLSTQRRKRNKGWSRDEGTEAEIRKVMNGDYQTSYVEVKRGSKIGEKSAWMLNLSIDVPKIDKGVDPSIIGGIDVGVKSPLVCAINNAFSRYSISDNDLFHFNKKMFARRRILLKKTRHKRAGHGAKNKLKPISILTGKSERFRKKLIERWACEIADFFIKNKVGTVQMENLESMKRKEDSYFNIRLRGFWPYAEMQNKIEFKLKQYGIEIRKVAPNNTSKTCSKCGHLNNYFNFEYRKKNKFPHFKCEKCNFKENADYNAALNISNPKLKSTKEEP

SEQ ID NO: 2771 - protein, 726 aa, synthetic construct
SEVEFSHEYWMRHALTLAKRARDEREVPVGAILVLNNRVIGEGWNRAIGLHDPTAHAEIMALRQGGLVMRNYRLVDATLYVTFEPCVMCAGAMIHSRIGRVVFGVRNNKHGAAGSLVNVLNYPGMGHRVEITEGILADECAALLCDFYCMPRQVFNAQKRAQSSINSGGLSGGSSGSDTPGTSESATPESSGGGSSGSAKNTITKTLQLRIVRPYNSAEVEKIVADEKNNREKIALEKNKGKVKEACSKHLEVAAYCTTQVERNACLFCKARKLDDKFYQKLRGQFPDAVFWQELGEIFRQLQRQAAEIYNQSLIELYYEIFIKGKGFANASSVEHYLSDVCYTRAAELFKNAAIASGLRGKVKSNFRLKELKNMKSGLPTTKSDNFPIPLVKQKGGQYTGFEISSHNDDLVIKIPFGRWRVKREIDKYRPWEKFDFEQVRKSPQPISLLLSTQRRKRNKGWSEDEGTEAEIRKVMNGDYQTSYIEVKRGSKTGEKSAWMLNLSIDVPKIDKGVDPSIIGGIDVGVKSPLVCAINNAFSRYSISDNDLFHFNKKMFARRRILLKKNRHRRAGHGAKNKLKPISILTEKSKRFRKKLIERWACEIADFFIKNKVGTVQMENLESMKRKEDSYFNIRLRGFWPYAEMQNKIEFKLKQYGIEIRKVAPNNTSKTCSKCGHLNNYFNFEYRRKNKFPHFKCEKCNFKEDADYNAALNISNPKLKSTKEEP

SEQ ID NO: 2772 - protein, 726 aa, synthetic construct
SEVEFSHEYWMRHALTLAKRAHDEREVPVGAVLVLNNRVIGEGWNRAIGLHDPTAHAEIMALRQGGLVLQNYRLVDATLYVTFEPCVLCAGAMVHSRIGRVVFGARNSKRGAAGSLMNILNYPGMNHRVEITEGILADECAALLCDFYRMPRQVFNAQKKAQSSINSGGSSGGSSGSETPSTSESATPESSGGSSGGSAKNTITKTLQLRIVRPYNSAEVEKIVTDEKNNREKIALEKNKDKVKEACSKHLKVASYCTTQVERNACPFCKARKLDDKFYQKLRGQFPNAVFWQELGEILRQLQKQAAEIYNQSLIELYYEIFIKGRGFANASSVEHYLSDVCYTRAAELFKNAAIASGLRGKVKSNFRLKELKNMKSGLPTTKSDNFPIPLVKQKGGQYTGFEISSHNDDFIIKIPFGRWQVKEEIDKYRPWEKFDFEQVRKNPKPISLLLSIQRRKRNKGWSRDEGTEAEIRKVMNGDYQTSYIEVKRGSKIGEKSAWMLNLSIDVPKIDKGVDPSIIGGIDVGVKSPLVCAINNALSRYSISDNDLFHFNKKMFARRRILLKKNRRKRAGHGAKNKLKPISILTGKSERFRKKLIERWACEIADFFIKNKVGTVQMENLESMKRKEDSYFNIRLRGFWPYAEMQNKIEFKLKQYGIEIRKVAPNNTSKTCSRCGHLNNYFNFEYRKKNKFPHFKCEKCNFKENADYNAALNISNPKLKSTKEEP

SEQ ID NO: 2773 - protein, 726 aa, synthetic construct
SEVEFSHEYWMRHALTLAKRARDRREVPVGAVLVLNNRVIGEGWNRAIGLHDPTAHAEIMALRQGGLVMQNYRLIGATLYVTFEPCVMCAGAMIHSRIGRVVFGVRNNKHGAAGSLVNVLDYPGMNHRVEITEGILADECAALLCDFYRMPRQVFNARKKAQSSISPGGSSGGSSGSEAPGTSESATPESSGGSSGGSAKNTITKTLKLRIVRPYNSAEVEKIVADEKNNREKIALEKNKDKVKEACSKHLKVATYCTTQVERNACLFCKARKLDDKFYQKLRGQFPDAVFWQEVGEIFRQLQKQAAEIYNQSLIELYYEIFIKGKGIANASSVGHYLSDVCYTRAAELFKNAAIASGLRGKVKSNFRLKELKNMKSGLPTTKSDNFPIPLVKQKGGQYTGFEISSHNDDFIIKIPFGRWQVKKEIDKYRPWEKFDFEQVRKSPKPISLLLSTQRRKRNKGWSKDEGTEAEIRKVMNGDYQTSYIEVKRGSKIGEKSTWMLNLSIDVPKIDKGVDPNIIGGIDVGVKSPLVCAINNALSRYSISDNDLFRFNKKMFARRRILLKKNRHRRAGHGAKNKLKPIAVLAEKSEGFRKKLIERWACEIADFFIKNKVGTVQMENLESMKRREDSYFNIRLRGFWPYAEMQNKIEFKLKQYGIEIRKVAPNNTSKTCSKCGHLNNYFNFEYRKKNKFPHFRCEKCNFKENADYNAALNISNPKLKSTKEEP

SEQ ID NO: 2774 - protein, 726 aa, synthetic construct; identical to SEQ ID NO: 684

SEQ ID NO: 2775 - protein, 726 aa, synthetic construct
SEVEFSHEYWMRHALTLAKRARDEREVPVGAVLVLNNRVIGVGWNRAIGLHDPTAHAEIMALRQGGLVTQNYRLIDATLYVTFEPCVMCAGAMIHSRIGRVVFGVRNNKHGAAGSLMNVLNYPGMNHRVEITEGILADECAALLCDFYRMPRQVFNARKKAQSSINPGGSSGGSSGSKTPGTSESATPESSGGSSGGSAKNSITKTLKLRIVRPYNSAEVEKIVADEKNNREKIALEKNKGKVKEACSKHLKVAAYCTTQVERDACLFCKARRLDDKFYQKLRGQFPDAVFWQEIGEIFRQLQKQAAETYNQSLIELYYEIFIKGKGFANASSVEHYLSDVCYTRAAELFKNAAIASGLRGKVKSNFRLKELKNMKSGLPTTKSDNFPIPLVKQKGGQYTGFEISSHNDDFIIKIPFGRWQVKKEISKHRPWEKFDFEQVRKSPKPISLLLSTQRRKRNRGWSKDEGTEAEIKKVMNGDYQTSYIEVKRGSKIGEKSAWMLNLSIDVPKIDKGVDPSIIGGIDVGVKSPLVCAINNAFSRYSISDNDLFHFNKKMFARRRILLKKSKHRRAGHGAKSKLKPITILTEKSGRFRKKLIERWACEIADFFIKNKVGTVQMENLESMKRKEDSYFNIRLRGFWPYAEMQNKIEFKLKQYGIEIRKVAPNNTSKTCSKCGHLNNYFNFEYRKRNKFPHFKCEKCNFKENADYNAALNISNPKLKSTKEEP

SEQ ID NO: 2776 - protein, 726 aa, synthetic construct
SEVEFSHEYWMRHALTLAKRARDEREVPVGAVLVLNNRVIGEGWNRAIGLHDPTAHAEIMALRQGGLVMQNYRLTDATLYVTFEPCVMCAGAMIHSRIGRVVFGVRNSKRGAAGSLMNVLNYPGMNHRVEITEGILVDECAALLCDFYRMPCQVLNAQKKAQSSISSGGSSGGSSGGDTLGASESVTPKSSVGSSASSTKNTITKTLKLRIVRPYNSAEVEKIVADEKDNREKIALEKNKDKVKEACSKHLKVAAYCTTQVERNACQFCKARKLDDKFYQKLRGQFPDAVFWQEIGEIFRQLQKQAAEIYNQSLVELYYEIFIKGKGFANASSAEHYLSDVCYTRAAELFKNAAIASGLRGKVKSNFRLKELKNMKSGLPTTKSDNFPIPLVKQKGGQYTGFEISSHNDDFIIKIPFGRWQVKKEIDKYRPWEKFDFEQVRKSPKPISLLLSTQRRKRNKGWSKDEGTEAEIRKVMNGDYQTSYIEVKRGGKIGEKSAWMLNLSIDVPKIDKGVDPSIIGGIDVGVKSPLVCAINNAFSRYSISDNDLFRFNKKMFARRRILLKKNRHKRAGHGAKNKLKPITILTGKSRRFRKKLIERWACEIADFFIKNKVGTVQMESLESMKRKEDSYFNIRLRGFWPYAEMQNKIEFKLKQYGIKIRKVAPNNTSKTCSKCGHLNNYFSFEYRKKNKFPHFKCEKCNFKENADYNAALNISNPKLMSTKEEP

SEQ ID NO: 2777 - protein, 726 aa, synthetic construct
SEVEFSHEYWMRHALTLAKRARDEREVPVGAILVLNNRVIGEGWNRAIGLHDPTAHAEIMALRQGGLVMQNYRLIDATLYVTFEPCVMCAGAMVHSRIGRVVFGVRNSKRGAAGSLMNVLDYPGMGHRVEITEGILADECAALLCDFYCMPRQVFNAQKRAQSSISSGGSSGGCSGSEMPGASESVTPKSSGGSSAGSTKNTITKTLKLRIVRPYNSAEVEKIVADEKNSREKIALERNKDKVKEACSKHLKVAAYCTTQVERNACLFCKARKLDDKFYQKLRGQFPDAVFWQEVGEIFRQLQKQAAEIYNQSLVELYYEILIKGKGIANASSVEHYLSDVCYTRAAELFKNAAIASGLRNKIKSNFRLKELRNMKSGLPTTKSDNFPIPLVRQKGGQYTGFEISNYNGDFIIKIPFGRWQVKKEIDKYRPWEKFDFEQVRKSPKPISLLLSTQRRKRNKGWSKDEGTEAEIRKVMNGDYQTSYIEVKRGSKTGEKSAWMLNLSIDVPKIDKGVDPCIIGGIDVGVKSPLVCAINNAFSRYSISDNDLFHFNKKMFARRRILLKENGRKRAGHGAKNKLKPITIMTEKSKRFRKKLIERWACEIADFFIKNKVGTVQMENLESMKRKEDSYFNIRLRGFWPYAEMQNKIEFKLKQYGIVVRKVAPNNTSKTCSKCGHLNNYFNFEYRKKNKFPHFKCEKCNFKEDADYNAALNISNPKLKSTKEEP

SEQ ID NO: 2778 - protein, 726 aa, synthetic construct
GEVGFSHEYWMRRALTLAKRARDEREVPVGAILVLNNRVIGEGWNRAIGLHDPTAHAEITALRQGGLVMQNYRLIDATLYVTFEPCVMCAGAMIHSRIGRVVFGVRNSKHGAAGSLVNVLNYPGMNHRVEITEGILADECAALLCDFYRMSRQVFNARKKAQPSINPGGSSGGSSGSETPGTSESATPESSGGSSGGSAKNTITKTLKLRIVRPYNSAEVEKIVADEKNNREKIALEKNKDKVKEACSKHLKVAAYCTTQVERNACLFCKARRLDDKFYQKLRGQFPDAVFWQEIGEIFRQLQKQAAEIYNQSLIELYYEIFIKGKGIANASSVEHYLSDVCYTRAAELFKNAAIASGLRNKVKSNFRLKELRSMKSGLPTTKSDNFPIPLVRQKGGQYTGFEISNHNSDFIIKIPFGRWQAKKEIDKYRPWEKFDFEQVRKSPKPISLLLSTQRRKRNRGWSKDESTEAEIKKVMNGDYQTSYIEVKRGSKVGEKSTWMLNLSIDVPKIDKGVDPSIIGGIDVGVKSPLVCAINNAFSRYSISDNDLYRFNKKMFARRRILLKKNRRKRAGHGAKNKLKPISILTEKSERFRKKLIERWACEIADFFVKNKVGTVQMENLESMKRKEDSYFNIRLRGFWPYAEMQNKIELKLKQYGIVIRKVAPNNTSKTCSMCGHLNNYFNFEYRKKNKFPHFKCEKCNFKEDADYNAALNISNPKLKSTKEEP

SEQ ID NO: 2779 - protein, 726 aa, synthetic construct
SEVESSHEYWMRHALTLAKRARDEREVPVGAILVLNNRVIGEGWNRAIGLHDPTAHAEIMALRQGGLVMQNYRLIDATLYVTFEPCVMCAGAMIHSRIGRVVFGVRNSKHGAAGSLVNVLNYPGMNHRVEITEGILADECAALLCDFYRMPRQVFNARRKAQSSINPSGSSGGSSGSVTPGTSESATQESSGGSSGGSAKNTITKTLKLRIVRPYNSAEVEKIVADEKNNREKIALEKNKDKVKEACSKHLKVAAYCTTQVERNACLFCKARKLDDKFYQKLRGQFPDAVFWQEIGEIFRQLQKQAAEIYNQSLIELYYEIFIKGKGFANASSVEHYLSDVCYTRAAELFKNAAIASGLRGKVKSNFRLKELKNMKSGLPTTKSDNFPIPLVRQKGGQYTGFEISSHNDDFIIKIPFGRWQVKKEIDKYRPWEKFDFEQVRKSPKPISLLLSTQRRKRNKGWSKDEGTEAEIRKVMNGDYQTSYIEVKRGSKTGEKSAWMLNLSIDVPKIDKGVDPSIIGGIDVGVKSPLVCAINNAFSRYSISDNDLFHYNKKMFARRRILLKKNRHKRAGHGAKNKLKPISILTEKGKRFRKKLIERWACEIADFFIKNKVGTVQMENLESMKRKEDSYFNIRLRGFWPYAEMQNKIEFKLKQYGIEIRKVAPNNTSKTCSKCGHLNSYFNFEYRKKNKFPHFKCEKCNFKENADYNAALNISNPKLKSTKEEP

SEQ ID NO: 2780 - protein, 726 aa, synthetic construct
SEVEFSHEYWMRHALTLAKRARDEREVPVGAVLVLNNRVIGEGWNRAIGLHDPTAHAEIMALRQGGLVMQNYRLIDATLYVTFEPCVMCAGAMVHSRIGRVVFGVRNSKRGAAGSLMNVLDYPGMGHRVEITEGILADECAALLCDFYRMPRQVLNAQKKAQSSINPSGSSGGSSGGKAPGTSESATLESSGGSSGGSAKNSITKTLKLRIVRPYNSAEVEKIVADEKNNREKIALEKNKDKVKEACSKHLKMASYCTTQVERNACLFCKARKLDDKFYQKLRGQFPDAVFWQELGEIFRQLQKQAAEVYNQSLVELYYEILIRGKGIANASSVEHYLSDVCYTRAAELFKNAAIASGLRNKIKSNFRLKELKNMKSGLPTTKSDNFSIPLVKQKGGQYTGFEISSHNDDFIIKIPFGRWQVKKEIDKYRPWEKFDFEQVRKNPKPISLLLSIQRRKRNKGWSRDEGTEAEIRKVMNGDYQTSYIEVKRGSKIGEKSAWMLNLSIDVPKIDKGVDPSIIGGIDVGVKSPLICAINNAFSRYGICDNDLFRFNKKVFARRRILLKKNRHKRAGHGTKNKLKPITILTEKSGRFRKKLIERWACEIANFFIKNKVGTVQMENLESMKRKEDSYFNIRLRGFWPYAEMQNKIEFKLRQYGIKIRKVAPNNTSKTCSKCGHLNNYFSFEYRKKNKFPHFKCEKCNFKEDADYNAALNISNPKLKSTKEEP

SEQ ID NO: 2781 - protein, 726 aa, synthetic construct
SEVEFSHEYWMRHALTLAKRARDEREVPVGAILVLNNRVIGEGWNRAIGLHDPTAHAEIMALRQGGLVMQNYRLIDATLYVTFEPCVMCAGAMIHSRIGRVVFGVRNSKRGAAGSLMNVLNYPGMNHCVEITEGILVDECAALLCDFYRMPRQVLNAQKKAQSSISSGGSSGGSSGSETPGASESATPKSSGGSSAGSTKNTITKALKLRIVRPYNSAEVEKIVADEKNNRERIALEKNKDKVKEACSKHLKVAAYCTTQVERNACLFCKARKLDDKFYQKLRGQFPDAVFWQETGEIFRQLQRQAAEIYNQSLIELYYEIFIKGKGFANASSVEHYLSDVCYTRAAELFKNAAIASGLRGKVKGNFRLKELKNMKSGLPTTKSDNFPIPLVKQKGGQYTGFEISSHNDDFIIKIPFGRWQAKKEIDKYRPWEKFDFEQVRRSPKPISLLLSTQRRKGNKGWSKDEGTEAEIRKVMNGDYQTSYIEVKRGSKIGEKSAWMLNLSIDVPKIDKGVDPSIIGGIDVGVKSPLVCAINNAFSRYSISDNDLFHFNKKMFARRRILLKKNRHKRAGHGAKNKLKPISILTEKSKRFRKKLIERWACEIADFFIKNKVGTVQMENLESMKRKEDSYFNIRLRGFWPYAEMQNKIEFKLKQYGIEIRKVAPNNTSKTCSKCGHLNNYFNFEYRRKNKFPHFKCEECNFKEDADYNAALNISNPKLKSTKEEP

SEQ ID NO: 2782 - protein, 726 aa, synthetic construct
SEVEFSHEYWMRHALTLAKRARDEREVPVGAILVLNNRVIGEGWNRAIGLHDPTAHAEIMALRQGGLVMQNYRLIDATLYVTFEPCVMCAGAMIHSRIGRVVFGVRNNKHGAAGSLVNVLNYPGMNHRVEITEGILADECAALLCDFYRMPRQVFNARKKAQSSINPGGSSGGSSGSETPGTSESATPESSGGSSGSSAKNTITKTLKLRIVRPYNSAEVEKIVADEKNNRERIALEKNKNKVKEACSEHLKVAAYCTTQVERSACLFCKARKLDDKFYQELRGQFPDAVFWQEIGEIFRQLQKQAAEIYNQSLIELYYEIFIKGKGFANASSVEHYLSDVCYTRAAELFKNAAIASGLRGKVKSNFRLKELKNMKSGLPTTKSDNFPIPLVKQKGGQYTGFEISSHNDDFIIKIPFGRWQVKEEIDKYRPWEKFDFEQVRKNPKPISLLLSVQRRKRNKGWSRDEGTEAEIRKVMNGDYQTSYIEVKRGSKIGEKSAWMLNLSIDVPKIDKGVDPSVIGGIDVGVKSPLICAINNAFSRYGISDNDLFRFNKKVFARRRILLKKNRHKRAGHGTKNKLKPITILTEKSGRFRKKLIERWACEIADFFIKNKVGTVQMENLESMKRKEDSYFNIRLRGFWPYAEMQNKIEFKLKQYGIKIRKVAPNNTSRTCSECGHLNNYFSFEYRKKNKFPHFKCEKCNFKEDADYNAALNISNPKLKSTKEEP

SEQ ID NO: 2783 - protein, 726 aa, synthetic construct
SEVEFSHEYWMRHALTLAKRARDEREVPVGAVLVLNNRVIGEGWNRAIGLHDPTAHAEIMALRQGGLVMQNYRLIDATLYVTFEPCVMCAGAMVHSRIGRVVFGVRNSKRGAAGSLMNVLDYPGMDHRVEITEGILADECAALLCDFYRMPRQVFNAQKKAQSSINSGGSSGGSSSSETPGTSESATSESSGGSSAGSTKDTITKTLKLRIVRPYNSAEVEKVVADEKNNREKIAMEKNKDKVREACSKHLKVASYCTTQVERNACLFCKARKLDDKFYQKLRGQFPDAVFWQELGGIFRQLQKQAAEIYNQSLIELYYEIFIKGKGITNASNVEHYLSDVCYTRAAELFKNAAIASGLRGKVKSNFRLKELKNMRSGLPTTKSDNFPIPLVKQKGGQYAGFEISSHNDDFIIKIPFGRWQVKKEIDKYRPWEKFDFGQVRKSPKPISLLLSTRRRKRNKGWSKDEGTEAEIRKVMNGDYQTSYIEVKRGSKIGEKSAWMLSLSIDVPKIDKGVDPSIIGGIDVGVKSPLVCAINNAFGRHSISDNDLFHFNKKMFARRRILLKKNRHKRAGHGAKNKLKPITVLTEKSVRFRKKLIERWACEIADFFIKNKVGTVQMENLESMKRKEDSYFNIRLRGFWPYAEMQNKIEFKLKQYGIEIRKVAPNNTSKTCSKCGHLNNYFSFEYRKKNKFPHFKCEKCNFKENADYNAALNISNPKLKSTKEEP

SEQ ID NO: 2784 - protein, 726 aa, synthetic construct
SEVEFSHEYWMRHALTLAKRARDEREVPVGAILVLNNRVIGEGWNRAIGLHDPTAHAEIMALRQGGLVMQNYRLIDATLYVTFEPCVMCAGAMIHSRIGRVVFGVRNSKHGAAGSLVNVLNYPGMNHRVEITEGILADECAALLCDFYRMPRQVFNARKKAQSSISSGGSSGGCSGSEMPGASESVTPKSSGGSSAGSTKNAITKTLKLRIVRPYNSAEVEKIVADEKNSREKIALEKNKDKVKEACSEHLKVAAYCTTQVERNACLFCKARKLDDRFYQKLRGQFPDAVFWQETGEIFRQLQRQAAEIYNQSLIELYYEIFIKGKGFANASSVEHYLSDVCYTRAAELFKNAAIASGLRGKVKSNFRLKELKNMKSGLPTTKSDNFPIPLVKQKGGQYTGFEISSHNDDFIIKIPFGRWQVKKEIDKYRPWEKFDFEQVRKSPKPISLLLSTQRRKRNKGWGKDGGTEAEIRKVMNGDYQTSYIEVKRGSKTGEKSAWMLNLSIDVPKIDKGVDPSIIGGIDVGVKSPLVCAINNAFSRYSISDNDLFRFNKKMFARRRILLKKNRHRRAGHGAKNKLKPISILTEKSKRFRKKLIERWACEIADFFIKNKVGTVQMENLESMKRKEDSYFNIRLRGFWPYAEMQNKIEFKLKQYGIEIRKVAPNNTSKTCSKCGHLNNYFNFEYRKKNKFPHFKCEKCNFKENADYNAALNISNPMLKSTKEEP

SEQ ID NO: 2785 - protein, 726 aa, synthetic construct
SEVEFSHEYWMRHALTLAKRARDEREVPVGAILVLNNRVIGEGWNRAIGLHDPTAHAEIMALRQGGLVMQNYRLIDATLYVTFEPCVMCAGAMIHSRIGRVVFGVRNNKHGAAGSLVNVLNYPGMNHRVEITEGILADECAALLCDFYRMPRQVFNARKKAQSSINPGSPSGGSSGSETPDTSESATPESSGGSSGGSAKNTITKTLKLRIVRPYNSTEVEKIVADEKNNREKIALEKNKDKVKEACSKHLKVAPYCTTQVERNACLFCKARKLDDKFYQKLRGQFPNAVFWQELGEIFRQLQKQAAEIYNQSLIELYYEIFIKGKGFANASSVEHYLSDVCYTRAAELFKNAAIASGLRGKVKSNFRLKELKNMKSGLPTTKSDNFPIPLVKQKGGQYTGFEISSHNDDFIIKIPFGRWQAKKEINKHRPWEKFDFEQVRKSPKPISLLLSTQRRKRNKGWSKDEGTEAEIRKAMNGDYQTSYIEVKRGSKIGEKSAWMLSLSIDVPKIDKGVDPRIIGGIDVGVKSPLVCAINNAFCRYSISDNDLFHFNKKMFARRRILLKKSRHKRAGHGAKNKLKPISILTEKSKRFRKKLIERWACEIADFFIKNKVGTVQMENLESMKRKEDSYFNIRLRGFWPYAEMQNKIEFKLKQYGIEIRKVAPNNTSKTCSKCGHLNNYFNFEYRKKNKFPHFKCEKCNFKENADYNAALNISNPKLKSTKEEP

SEQ ID NO: 2786 - protein, 726 aa, synthetic construct
SEVEFSHEYWMRHALTLAKRARDEREVPVGAVLVLNNRVIGEGWNRAIGLHDPTAHAEIMALRQGGLVMQNYRLIDATLYVTFEPCVMCAGAMIHSRIGRVVFGVHNNKHGAAGSLVNVLNYPGMNHRVEITEGILADECAALLCDFYRMPRQVFSARKKAQSCINPGGSSGGSSGSETPGTSESATPESSGGSSGSSAKNTITKTLKLRIVRPYNSAEVEKIVADEKNNREKIALEKNKDKVKEACSKHLKVAAYCTTQVGRNACLFCKARRLDDKFYQKLRGQFPDAVFWQEIGEIFRQLQKQAAEVYNQSLVELYYEILIKGKGTANASSVEHYLSDVCYTRAAELFKNAAIASGLRSKIKSNFRLKELRNMKSGLPTTKSDNFPIPLVRQKGGQYTGFEISSHDGDFIIKIPFGRWQVKKEINKHRPWEKFDFEQVRKSPKPISLLLSTQRRKKNKGWSKDEGTEAEIRRVMNGDYQTSYIEVKRGSKIGEKSAWMLNLSIDVPKIDKGVDPSIIGGIDVGVKSPLVCAINNSSSRYSICDNDLFRFNKKMFARRRILLKKNRHKRAGHGAKNKLKPITILTKKSERFRKKLIERWVCEVADFFIKNKVGTVQMENLESMKRKEDSYFNIRLRGFWPYAEMQNRIELKLKQYGIEIRRVAPNNTSRTCSKCGHLNNYFNFEYRKKSKFPHFKCEKCNFREDADYNAALNISNPKLKSTKEEP

SEQ ID NO: 2787 - protein, 726 aa, synthetic construct
SEDEFSHEYWMRHALTLAKRARDGREVPVGAVLVLNNRVIGEGWNRAIGLHDPTAHAEIMALRQGGLVMQNYRLINATLYVTFEPCVMCAGAMIHSRIGRVVFGVRNSKHGAAGSLMNVLNYPGMNHRVEITEGILADECAALLCDFYRMPRQVFSARKKAQSSINSGDSSGGSSGSETPGASESATPKSSGGSSAGSTKDTITKTLKLRIVRPYNSAEVEKIVADEKNSREKIALEKNKDKVKEACSKHLKVASYCTTQVERNACLFCKARKLDDKFYQKLRGQFPDAVFWQEIGEIFRQLQKQAAEIYNQSLIELYYEIFIKGKGFANASSAEHYLSDVCYTRAAELFKNAAIASGLRGKVKSNFRLKELKNMKSGLPTTKSDNFPIPLVKQKGGKYTGFEISRHNDDFIIKIPFGRWQVKKETDKYRPWEKFDFEQVRKSPKPISLLLSTRRRKRNKGWSKDEGTEAEIRRVMNGDYQTSYIEVKRGSKIGEKSAWMLSLSIDVPKIDKGVDPRIIGGIDVGVKSPLVCAINNVLSRYSISDNDLFHFNKKMFARRRILLKKNGHKRAGHGAKNKLKPITIMTEKSKRFRKKLIERWACEIADFFIKNKVGTVQMENLESMKRKEDSYFNIRLRGFWPYAEMQNKIEFKLKQYGIVVRKVAPNNTSKTCSQCGHLNNYFNFEYRKKNKFPYFKCEKCNFKENADYNAALNISNPQLKSTKGEP

SEQ ID NO: 2788 - protein, 726 aa, synthetic construct
SEVEFSHEYWMRHALTLAKRARDEREVPVGAVLVLNNRVIGEGWNRVIGLHDPTAHAEIMALRQGGLVMQNYRLTDATLYVTFEPCVMCAGAMIHSRIGHVVFGVRNSKRGAAGSLMNVLNYPGMNHCVEITEGILVDECAALLCDFYRMPRQVLNAQKKAQSTINSGSSSGGSSGSETPGTSESPTPESSGGSPGGSAKNTITKTLKLRIVRPYNSAEVEKIVADEKNNREKIALEKNKDKVKEACSKHLKVAAYCTTQVERNACLFCKARKLDDKFYQKLRGQFPDAVFWQEIGEIFRQLQKQAAEIYNQSLIELYYEIFIKGKGFANASSVEHYLSDVCYTRAAELFKNAAIASGLRGKVKSNFRLKELKNMKSGLPTTKSDNFPIPLVKQKGGQYTGFEISSHNDDFIIKIPFGRWQVKEEIDKYRPWEKFDFEQVRKNPKPISLLLSTQRRKRNKGWSKDEGTEAEIRKVMNGDYQTSYIEVKRGSKTGEKSAWMLNLSIDVPKIDKGVDPSIIGGIDVGVKSPLVCAINNAFSRYSISDNDLFHFNKKMFARRRILLKKTRHKRAGHGAKNKLKPISILTEKSERFRKKLIERWACEIADFFIKNKVGTVQMENLESMKRREDSYFNIRLRGFWPYAEMQNKIEFKLKQYGIEIRKVAPNNTSKTCSKCGHLNNYFNFEYRKKNKFPHFKCEKCNFKENADYNAALNISNPKLKSTKEEP

SEQ ID NO: 2789 - protein, 726 aa, synthetic construct
SEVEFSHEYWMRHALTLAKRARDEREVPVGAILVLNNRVIGEGWNRTTGLHDPTAHAEIMALRQGGLVMQNHRLVDATLYVTFEPCVMCAGAMIHSRIGRVVFGVRNSKRGAAGSLTNVLNYPGMNHRVEITEGILVDECAALLCDFYRMPRRVFNAQKRAQSTINTGGSTGSSSGSETPGTSESPTPESSGGSPGGSAKNTITKTLKLRIVRPYNSAEVEKIVADEKNNREKIALEKNKDKVKEACSKHLKVAAYCTTQVERNACLFCRARKLDDKFYQKLRGQFPDAVFWQEIGEIFRQLQKQAAEIYNQSLIELYYEIFIKGKGFANASSVEHYLSDVCYTRAAELFKNAAIASGLRNKIKSNFRLKELRNMKSGLPTTKSDNFPIPLVRQKGGQYTGFEISNHNSDFIIKIPFGRWQAKKEIDKYRPWEKFDFEQVRKSPKPISLLLSTQRRKRNRGWSKDEGTEAEIRKVMNGDYQTSYIEVKRGSKIGEKSAWMLNLSIDVPKIDKGVDPSIIGGIDVGVKSPLVCAIDNALSRYSISDNDLFHFNKKMFARRRILLKKNRHRRAGHGARNKLKPITVLTEKSKRFRKKLIERWACEIANFFIKNKVGTVQMENLESMKRKEDSYFNIRLRGLWPYAEMQNKIEFKLKQYGIEIRKVAPNNTSKTCSKCGHLNNYFNFEYRKRNKFPHFKCEKCNFKENADYNAALNISNPKLKSTKEEP

SEQ ID NO: 2790 - protein, 726 aa, synthetic construct
SEVEFSHEYWMRHALTLAKRARDEREVPVGAVLVLNNCVIGEGWNRAIGLHDPTAHAEIMALRQGGLVMQNYRLSDATLYVTFEPCVMCAGAMVHSRIGRVVFGVRNSKRGAAGSLMNVLDYPGMGHRVEITEGILADECAALLCDFYCMPRQAFSAQKRAQSSINSGGSSGGSSGSETPGTSESAAPESSGGSSGGSAKNTITKTLKLRIVRPYNSAEVEKIVADEKNNREKIALEKNKGKVKGACSEHLKVAAYCTTQVGRNACLFCKARKLDDKFYQKLRGQFPDAVFWQEIGEVFRQLQKQAAEIYNQSLIELYYEILIKGKGIANASSVEHYLSDVCYTRAAKLFKNAAIASGLRNKIKSNFRLKELRNMKSGLPTTKSDNFPIPLVRQKGGQYTGFEISNHDGDFIIKIPFGRWQVKKEIDKYRPWEKFDFEQVRKSPKPISLLLSTQRRKRNKGWSKDEGTEAEIRKVMNGDYQTSYIEVKRGSKTGEKSTWMLNLSIDVPKIDKGVDPSIIGGIDVGVKSPLVCAINNASSRYSISDNDLFRFNKKVFARRRILLKKNRHKRAGHGTKNKLKPITILTEKSGRFRKKLIERWACEIANFFIKNKVGTVQMENLESMKRKEDSYFNIRLRGFWPYAEMQNKIEFKLKQYGIKIRKVAPNNTSKTCSKCGHLNNYFGFEYRKKNKFPHFKCEKCNFKEDADYNAALNISNPKLKSTKEEP

SEQ ID NO: 2791 - protein, 726 aa, synthetic construct
SEVEFSHEYWMRHALTLAKRARDEREVPVGAILVLNNRVIGEGWNRAIGLHDPTAHAEIMALRQGGLVMQNYRLIDATLYVTFEPCVMCAGAMIHSRIGRVVFGVRNSKHGAAGSLVNVLNYPGMNHRVEITEGILADECAALLCDFYRMPRQVFNARKKAQSSINPSGSSGGSSGSVTPGTSESATPESSGGSFGGSAKNTITKTLQLRIVRPYNSAEVEKIVADEKNNRERIALEKNKDKVKEACSEHLKVAAYCTTQVERNACLFCKARKLDDRFYQKLRGQFPDAVFWQEIGEIFRQLQKQAAEIYNQSLIELYYEIFIKGKGFANASSVEHYLSDVCYTRAAELFKNAAIASGLRGKVKSNFRLKELKNMKSGLPTTKSDNFPIPLVKQKGGQYTGFEVSNHDSDFIIKIPFGKWQVKKEIDKYRPWEKFDFEQVRKSPKPISLLLSTQRRKRNKGWGKDEGTEAEIRKVMNGDYQTSYIEVKRGSKIGEKSAWMLNLSIDVPKVDKGVDPNIIGGIDVGVKSPLVCAINNALSRYSISDNDLFHFNKKMFARRRILLRKNRYKRAGHGARNKLKPITVLTEKSERFRKKLIERWACEIANFFIKSKVGTVQMEDLESMKRREDSYFNIRLRGFWPYAEMQNKIEFKLKQYGIEIRKVAPNNTSKTCSKCGHLNNYFNFEYRKMNKFPHFKCEKCNFKENADYNAALNISNPKLKSTKEEP

SEQ ID NO: 2792 - protein, 726 aa, synthetic construct
SEVEFSHEYWMRHALTLAKRARDGREVPVGAVLVLNNRVIGEGWNRAIGLHDPTAHAEIMALRQGGLVMQNYRLIDATLYVTFEPCVMCAGAMVHSRIGRVVFGVRNSKRGAAGSLMNVLDYPGMGHRVEITGGILADECAALLCDFYCMPRQVFSAQKRAQSSINSGGSSGGSSGSETPGTSESATPESSGGGSSGSAKNTITKTLQLRIVRPYNSAEVEKIVADEKNNREKIALEKNKDKVKEACSKHLKVAAYCTTQVERNACLFCKARKLDDKFYQRLRGQFPDAVFWQELGEIFRQLQKQAAEIYNQSLIELYYEIFIKGKGITNASRVEHYLSDVCYTRAAELFKNAAIASGLRSKVRSNFRLKELKNMKSGLPTTKSDNFPIPLVKQKGGQYTGFEISSHNDDFIIKIPFGRWQVKKEIDKYRPWEKFDFEQVRKSSKPISLLLSTQRRKRNKGWSKDEGTEAEIRKVMNGDYQTSYIEVKRGSKTGEKSAWMLNLSIDVPKIDKGVDPSIIGGIDVGVKSPLVCAINNAFSRYSISDNDLFRFNKKMFARRRILLKKNRHKRAGHGAKNKLKPISILTEKSERFRKKLIEKWACEIADFFVKNKVGTVQMENLESMKRKEDSYFNIRLRGFWPYAEMQNKIEFKLKQYGIKIRKVAPNNTSKTCSKCGHLNNYFNFEYRKKNKFPHFKCERCNFKENADYNAALNISNPKLKSTKEEP

SEQ ID NO: 2793 - protein, 726 aa, synthetic construct
SEVEFSHEYWMRHALTLAKRARDEREVPVGAVLVLNNRVIGEGWNRAIGLHDPTAHAEIMALRQGGLVMQNYRLVDATLYVTFEPCVLCAGAMVHSRIGRVVFGVRNSKRGAAGSLMNVLNYPGMNHRVEITEGILADECAALLCDFYRMPRQVFNARKRARSNINSGGSSGGSSGSETLGTREGATLESSGGSSGGSAKNTITKTLKLRIVRPYNSAEVEKIVADEKNNREKIALEKNKDKVKEACSEHLKVAAYCTTQVERNACLFCKARKLDDKFYQKLRGQFPDAVFWQEIGEIFRQLQKQAAEIYNQSLIELYYEIFIKGKGFANASSVEHYLSDVCYTRAAELFKNAAIASGLRNKTKSNFRLKELRSMKSGLPTTKSDNFPIPLVKQKGGQYTGFEISNHNSDFIIKIPFGRWQAKKEIDKYRPWEKFDFEQVRKSPKPISLLLSTQRRKRNKGWSKDEGTEAEIRKVMNGDYQTSYIEVKRGSKIGEKSAWMLNLSIDVPKIDKGVDPSIIGGIDVGVKSPLVCAINNALSRYSISDNDLFHFNKKMFARRRILLKKNRHRRAGHGAKNKLKPIAVLAEKSEGFRKKLIERWACEVADFFIKNKVGTVQMENLESMKRREDSYFNIRLRGFWPYAEMQNKIEFKLRQYGIEIRKVAPNNTSKTCSKCGHLNNYFDFEYRKKNKFPHFKCEKCNFRENADYNAALNISNPKLRSTKEEP

SEQ ID NO: 2794 - protein, 726 aa, synthetic construct
SEVEFSHEYWMRHALTLAKRARDEREVPVGAVLVLNNRVIGEGWNRAIGLHDPTAHAEIMALRQGGLVLQNYRLVDATLYVTFEPCVLCAGAMVHSRIGRVVFGARNSKRGAAGSLMNILNYPGMNHRVEITEGILADECAALLCDFYRMPRQVFNAQKKAQSSINSGGSSGGSSGSETPSTSESATPESSGGSSGGSAKNTITKTLQLRIVRPYNSAEVEKIVTDEKNNREKIALEKNKDKVKEACSKHLKMASYCTTQVERNACLFCKARKLDDKFYQKLRGQFPDAVFWQEIGEIFRQLQKQAAEVYNQSLVELYYEILIKGKGIANASSVEHYLSDVCYTRAAELFKNAAIASGLRNKIKSNFRLKELRNMKSGLPTTKSDNFPIPLVRQKGGQYTGFEISSHNDDFIIKIPFGRWQAKKEIDKYRPWEKFDFEQVRKSPKPISLLLSTQRRKRNKGWSKDEGTEAEIRKVMSGDYQTSYIEVKRGSKIGEKSAWMLNLSIDVPKIDKGVDPSIIGGIDVGVKSPLVCAINNAFSRYSISDNDLFHFNKKMFARRRILLKKNRHKRAGHGAKNKLKPISILTEKSKRFRKKLIERWACEIADFFIKNKVGTVQMENLESMKKKEDSYFNIRLRGFWPYAEMQNKIEFKLKQYGIEIRKVAPDNTSKTCSKCGHLNNYFNFEYRRKNKFPHFKCEKCNCKEDADYNAALNISNPKLKSTKEEP

SEQ ID NO: 2795 - protein, 726 aa, synthetic construct
SEVEFSHEYWMRHALTLAKRARDEREVPVGAVLVLNNRVIGEGWNRAIGLHDPTAHAEIMALRQGGLAMQNYRLVDATLYVTFEPCVLCAGAMVHSRIGRVVFGVRNNKHGAAGSLVNVLNYPGMNHRVEITEGILADECAALLCDFYRMPRQVFNARKKAQSSISPGGSSGSSSGSETPGTSESPTPESSGGSPGGSAKNTITKTLKLRIVRPYNSAEVEKIVADEKNNREKIALEKNKDKVKEACSKHLKVAAYCTTQVERNACLFCKARKLDDKFYQKLRGQFPDAVFWQELGEIFRQLQKQTAEIYNQSLIELYYEIFIKGKGFANASSVEHYLSDVCYTRAAELFKNAAIASGLRGKVKSNLRLKELKNMRSGLPTTKSDNFPIPLVKQKGGQYTGFEISSHNDDFIIKIPFGRWQVKREIDKYRPWERFDFEQVRKSPKPISLLLSTQRRKRNKGWNKDEGTEAEIRKVMNGDYQISYIEVKRGSKIGEKSAWMLNLSIDVPKIDKGVDPSIIGGIDVGVKSPLVCAINNAFSRYSISDNDLFHFNKKMFARRRILLKKNRHKRAGHGAKNKLRPISILTEKSERFRKKLIEKWACEIADFFIKNKVGTVQMENLESMKRKEDSYFNIRLRGFWPYAEMQNKIEFKLKQYGIEIRKVAPNNTSKTCSKCGHLNNYFNFEYRKKNKFPHFKCEKCNFKENADYNAALNISNPKLKSTKEEP

SEQ ID NO: 2796 - protein, 726 aa, synthetic construct
SEVEFSHEYWMRHALSLAKRARDEREVPVGAVLVLNNRVIGEGWNRAIGLHDPTAHAEIMALRQGGLVMQNNRLTDATLYVTFEPCVMCAGAMIHSRIGRVVFGVRNSKRGAAGSLMNVLNYPGMNHCVEITEGILVDECAALLCDFYRMPRQVLNAQKKAQSSISPGGSSGGSSGSETPGASESVTPKSSGGSSGGSAKNTITKTLKLRIVRPYNSAEVEKIVADEKNNREKIALEKNRDKVKEACSKHLEVAAYCTTQVERNACLFCKARKLDDRFYQKLRGQFPDAVFWQEIGEIFRQLQKQAAEIYNQSLIELYYEIFIKGKGFANASSVEHYLSDVCYTRAAELFKNAAIASGLRGKVKSNFRLKELKNMKSGLPTTKSDNFPIPLVKQKGGQYTGFEISNHDSDFIIKIPFGRWQAKKEIDKYRPWEKFDFEQVRKSPKPISLLLSTQRRKKNRGWSKDEGTEAEIKKVMNGDYQTSYIEVKRGSKIGEKSAWMLNLSIDVPKIDKGVDPSIIGGIDVGVKSPLVCAISNAFSRYSISDNDLFHFNKKMFARRRILLKKSKHKRAGHGAKNKLKPITILTEKSRRFRKKLIERWACEIADFFIKNKVGTVQMENLESMKRREDSYFNIRLRGFWPYAEMQNKIEFKLKQYGIEIRRVAPNNTSRTCSKCGHLNNYFNFEYRKTNKFPHFKCEKCNFREDADYNAALNISNPKLKSTKEGP

SEQ ID NO: 2797 - protein, 726 aa, synthetic construct
SEVEFSHEYWMRHALTLAKRARDGREVPVGAVLVLNNRVIGEGWNRAIGLHDPTAHAEIMALRQGGLVMQNYRLTDATLYVTFEPCVMCAGAMVHSRIGRVVFGVRNSKRGAAGSLMNVLNYPGVNHCVEITEGILVDECAALLCDFYRMPRQVLNAQKKAQSSISSGGSSGGCSGSEMPGASESVTPKSSGGSSAGSAKNTITKTLQLRIVRPYNSAEVEKIVADEKNNREKIALEKNKDKVKEACSEHLKVAAYCTTQVERNACLFCKARKLDDKFYQKLRGQFPDAVFWQEIGEIFRQLQKQAAEIYNQSLIELYYEIFIKGKGFANASSVEHYLSDVCYTRAAELFKNAAIASGLRGKVKSNFRLKELKNMKSGLPTTKSDNFPIPLVKQKGGQYTGFEISSHHDDFIIKIPFGRWQVKKEIDKYRPWEKFDFEQVRKSPKPISLLLSTQRRKRNMGWSKDEGTEAEIRKVMNGDYQTSFIEVKRGSKIGEKSAWMLSLSIDVPKIDKGVDPSIVGGIDVGVKSPLVCAINNALGRYSISDNDLFHFNKKMFARRRILLKKNRHKRAGHGAKNKLKPISILTEKSKRFRKKLIERWACEIADFFIKNKVGTVQMENLESMKRKEDSYFNIRLRGFWPYAEMQNKIEFKLKQYGIEIRKVAPNNTSKTCSKCGHLNNYFNFEYRRKNKFPHFKCEKCNFKEDADYNAALNISNPKLKSTKEEP

SEQ ID NO: 2798 - protein, 726 aa, synthetic construct
SEVEFSHEYWMRHALTLAKRARDEREVPVGAILVLNNRVIGEGWNRAIGLHDPTAHAEIMALRQGGLVMQNYRLIDATLYVTFEPCVMCAGAMIHSRIGRVVFGVRNNKHGAAGSLVNVLDYPGMNHRVEITEGILADECAALLCDFYCMPRQVFSAQKKAQSSISSGGSSGGSSGSETPGASESATPKSSGGSSGGSAKNTITKTLKLRIVRPYNSAEVEKIVADEKNNREKIALEKNKGKVKEACSKHLEVAAYCTTQVERNACLFCKARKLDDKFYQKLRGQFPDAVFWQELGEIFRQLQKQAAEIYNQSLIELYYEIFIKGKGIASASRVGHYLSDVCYTRAAELFKNAAIASGLRSKIKSNFRLKELKNMKSGLPTTKSDNFPIPLVKQKGGQYTGFEISSHNDDFIIKIPFGRWQVKKEINKFRPWEKFDFEQVRKSPKPLSLLLSTQRRKRNKGWSRDEGTEAEIRKVMNGDYQTSYIEVKRGSKIGEKSAWMLNLSIDVPKIDKGVDPSIIGGIDVGVKSPLVCAINNAFSRYSISDNDLFHFNKKMFARRRILLKKTRHKRAGHGAKNKLKPISILTGKSERFRKKLIERWACEIANFFIKNKVGTVQMENLESMKRKEDSYFNIRLRGFWPYAEMQNKIEFKLKQYGIKIRKVAPNNTSKTCSKCGHLNNYFSFEYRKKNKFPHFKCEKCNFKEDADYNAALNISNPKLKSTKEEP

SEQ ID NO: 2799 - protein, 726 aa, synthetic construct
SEDEFSHEYWMRHALTLARRARDGREVPVGAVLVLNNRVIGEGWNRAIGLHDPTAHAEIMALRQGGLVMQNYRLIDATLYVTFEPCVMCAGAMVHSRIGRVVFGARNSKRGAAGSLMNVLDYPGMDHRVEITEGILADECAALLCDFYRMPRQVLSAQKKAQSSISSGGSSGGSSGSETPGASGSVTPKSSVGSSAGSTKNTITKTLKLRIVRPYNSAEVEKIVADEKNNREKIALEKNKDKVREACSKHLKVASYCTTQVERNACPFCKARKLDDKFYQKLRGQFPDAVFWQELGEILRQLQKQAAEVYNQSLIELYYEIFIKGRGFANASSVEHYLSDVCYTRAAELFKNAAIASGLRGKVKGNFRLKELKNMKSGLPTTKSDNFPIPLVKQKGGQYTGFEISSHNDDFIIKIPFGRWQVKKEIDKYRPWEKFDFEQVRKSPKPISLLLSTQRRKRNKGWSKDEGTEAEIRKVMNGDYQTSYIEVKRGSKIGEKSAWMLNLSIDVPKIDKGVDPSIIGGIDVGVKSPLVCAINNAFSRYSISDNDLFRFNKKMFARRRILLKKNRHKRAGHGAKNKLKPISILTEKSKRFRKKLIEKWACEIADFFIKNKVGTVQMENLESMKRREDSYFNIRLRGFWPYAEMQNKIEFKLKQYGIEIRKVAPNNTSKTCSRCGHLNNYFNFEYRRKNKFPHFKCEKCNFKENADYNAALNISNPKLKSTKEEP

SEQ ID NO: 2800 - protein, 726 aa, synthetic construct
SEVEFSHEYWMRHALTLAKRARDEREVPVGAVLVLNNRVIGEGWNRAIGLHDPTAHAEILALRQGGLVMQNYRLTDATLYVTFEPCVMCAGAMIHSRIGRVVFGVRNSKHGAAGSLMDVLNYPGMNHCVEITEGILVDECAALLCDFYRMPRQVLNAQKKAQSSISSGGPSGGSSCSETPGASESVTPKSSGGSSAGSTKNTITKTLKLRIVRPYNSAEVEKIVADEKNNREKIALEKNKGKVKEACSKHLKVAAYCTTQVERNACLFCKARRLDDKFYQKLRGQFPDAVFWQELGEILRQLQKQAAEIYNQSLIELYYEIFIKGRGFANASSVEHYLSDVCYTRAAELFKNAAIASGLRGKVKSNFRLKELKNMKSGLPTTKSDNFPIPLVKQKGGQYTGFEISSHNDDFIIKIPFGRWQVKKEIDKYRPWEKFDFEQVRKSPKPISLLLSTQRRKRNKGWSKDEGTEAEIRKVMNGDYQTSYIEVKRGSKIGEKSAWMLNLSIDVPKIDKGVDPSIVGGIDVGVKSPLVCAIDNALSRYSISDNDLFHFNKKMFARRRILLKKNRHRRVGHGAKNKLKPISILTEKSKRFRKKLIERWACEIADFFIKNKVGTVQMENLEGMKRKEDSYFNIRLRGFWPYAEMQNKIVFKLKQYGIEIRKVAPNNTSKTCSKCGHLNNYFNFEYRKMNKFPHFKCEKCNFKENADYNAALNISNPKLKSTREEP

SEQ ID NO: 2801 - protein, 726 aa, synthetic construct
SEVEFSHEYWMRHALTLAKRARDEREVPVGAVLVLNNRVIGEGWNRAVGLHDPTAHAEIMALRQGGLVMQNYRLIEATLYVTFEPCIMCAGAMIHSRIGRVVFGARNSKRGAAGSLMNVLNYPGMNHRVEITEGILADECAALLCDFYRMPRQVFNAQKKAQSSISSGGSSGGSSGSETPGASESVTPKSSVGSSAGSTKNTITKTLKLRIVRPYNSAEVEKIVADEKNNRERIALEKNKDKVKEACSKHLKVAAYCTTQVERNACLFCKARRLDDKFYQKLRGQFPDAVFWQEIGEIFRQLQKQAAEIYNQSLIELYYEIFIKGRGFANASSVEHYLSDVCYTRAAELFKNAAIASGLRGKVKGNFRLKELKNMKSGLPTTKSDNFPIPLVKQKGGQYTGFEISSHNDDFIIKIPFGRWQVKKEIDKYRPWEKFDFEQVRKSPKPISLLLSTRRRKRNKGWSKDEGTEAEIRKVMNGDYQTSYIEVKRGSKIGEKSAWMLNLSIDVPKIDKGVDPSIIGGIDVGVKSPLVCAINNAFSRYSISDNELFHFNKKMFARRRILLKKNRHKRAGHGAKNKLKPISVLTEKSERFRKKLIERWACEIADFFIKNKVGTVQMENLESMKRKEDSYFNIRLRGFWPYAEMQNRIEFKLKQYGIEIRKVAPNNTSKTCSKCGHLNNYFNFEYRKKNKFPHFKCEKCNFKEDADYNAALNISNPKLKSTKEEP

SEQ ID NO: 2802 - protein, 726 aa, synthetic construct
SEAEFSHEYWMRHALTLAKRARDEREVPVGAVLVLNNRVIGEGWNRAIGLYDPTAHAEIMALRQGGLVMQNYRLIDATLYVTFEPCVMCAGAMIHSRIGRVVFGVRNSKHGAAGSLMNVLNYPGMGHRVEITEGILADECAALLCDFYCMPRQVFNAQKRAQSSINSGGSSGGSSGSDTPGTSESATPESSGGGSSGSAKNTITKTLQLRIVRPYNSAEVEKIVADEKNNREKIALEKNKDKVREACSKHLKVASYCTTQVERNACPFCKARKLDDKFYQKLRGQFPDAVFWQELGEILRQLQKQAAEIYNQSLIELYYEIFIKGRGFANASSVEHYLSDVCYTRAAELFKNAAIASGLRGKVKGNFRLKELKNMKSGLPTTKSDNFPIPLVKQKGGQYTGFEISSHNDDFIIKIPFGRWQVKKEIDKYRPWEKFDFEQVRKSPKPISLLLSTQRRKRNKGWSKDEGTEAEIRKVMNGDYQTSYIEVKRGSKTGEKSAWMLNLSIDVPKIDKGVDPSIIGGIDVGVKSPLVCAINNAFSRYSISDNDLFRFNKKMFARRRILLRKNRHKRAGHGAKNKLRPISILTEKSGRFRKKLIERWACEIADFFIKNKVGTVQMENLESMKRKEDSYFNIRLRGFWPYAEMQDRIEFKLKQYGIEIRKVAPNNTSKTCSKCGHLNNYFNFEYRKKNKFPHFRCEKCNFKENADYNAALNISNPKLKSTKEEP

SEQ ID NO: 2803 - protein, 726 aa, synthetic construct
SEVEFSHEYWMRHALTLAKRARDEREVPVGAVLVLNNRVIGEGWNRAIGLHDPTAHAEIMALRQGGLVMQNYRLSDATLYVTFEPCVMCAGAMIHSRVGRVVFGVRNSKRGAAGSLMNVLNYPGMNHCVEITEGILVDECAALLCDFYRMPRQVLSAQKKAQSSISLGGSSGGSSGSETPGTSESATPESSGGSSGGSAKNTITKTLKLRIVRPYNSAEVEKIVADEKNSREKIALEKNKDKVKEACSKHLKVAAYCTTQVERNACLFCKARKLDDKFYQKLRGQFPDAVFWQEIGEIFGQLQKQAAEIYNQSLIELYYEIFIKGKGFANASSVEHYLSDVCYTRAAELFKNAAIASGLRGKVKSNFRLKELKSMKSGLPTTKSDNFPIPLVKQKGGQYTGFEISSHNDDFIIKIPFGRWQEKEEIDKYRPWEKFDFEQVRRSPKPISLLLSTQRRKKNKGWSKDEGTEAEIRKVMNGDYQTSYIEVKRGSKIGEKSAWMLNLSIDVPKIDKGVDPSIIGGIDVGVKSPLVCAINNAFSRYSISDNDLFHFNKKMFARRRILLKKNRRRRAGHGAKNKLKPITILTEKSVRFRKKLIERWACEIADFFIKNKVGTVQMENLESMKRKEDSYFNIRLRGLWPYAEMQNKIEFKLKQYGIKIRKVAPNNTSKTCSKCGHLNNYFNFEYRKRNKFPHFKCEKCNFKENADYNAALNISNPKLKGTKEEP

SEQ ID NO: 2804 - protein, 726 aa, synthetic construct
SEDEFSHEYWMRHALTLAKRARDGREVPVGAVLVLNNRVIGEGWNRAIGLHDPTAHAEIMALRQGGLVMQNYRLIDATLYVTFEPCVMCAGAMVHSRIGRVVFGVRNSKRGAAGSLMNVLDYPGMGHRVEITEGILADECAALLCDFYCMPRQVFNAQKRAQPSINSGGSSGGSSGSETPGTSESATPESSGGGSSGSAKNTITKTLKLRIVRPYNSAEVEKIVADEKNNREKIALEKNKDKVREACSKHLKVASYCTTQVERNACPFCKARKLDDKFYQKLRGQFPDAVFWQEIGEIFRQLQKQAAEIYNQSLIELYYEILIKGKGFANASSAEHYLSDVCYTRAAELFKNAAIASGLRGKVKSNFRLKELKNMKSGLPTTKSDNFPIPLVKQKGGKYTGFEISNHNSDFIIKIPFGRWQVKKEIDKYRPWEKFDFEQVRRSPKPISLLLSTQRRKRNKGWSKDEGTEAEIRKVMNGDYQTSYIEVKRGSKIGEKSAWMLNLSIDVPKIDKGVDPSIIGGIDVGVKSPLVCAINNAFSRYSISDNDLFHFNKKVFARRRILLKKNRHRRAGHGAKNKLKPITILTEKSKRFRKKLIERWACEIADFFIKNKVGTVQMENLESMKRKEDSYFNIRLRGFWPYAEMQNKIEFKLKQYGIKIRKVAPNNTSRTCSKCGHLNNYFSFEYRKKNKFPHFKCEKCNFKEDADYNAALNISNPKLKGTKEEL

SEQ ID NO: 2805 - protein, 726 aa, synthetic construct
SEVEFSHEYWMRHALTLAKRARDEREVPVGAVLVLNNRVIGEGWNRAIGLHDPTAHAEIMALHQGGLVMQNYRLIDATLYVTFEPCVMCAGAMVHSRIGRVVFGVRNSKHGAAGSLVNVLNYPGMNHRVEITEGILADECAALLCDFYRMPRQVFNARKKAQSSINPSGSSGGSSGSVTPGISESATPESSGGGFGGSAKNTITKTLQLRIVRPYNSAEVEKIVADEKNSREKIALEKNKDKVKEACSKHLKVASYCTTQVERNACLFCKARKLDDKFYQKLRGQFPDAVFWQELGEIFRQLQKQAAEIYNQSLIELYYEIFIKGKGLANASSVEHYLSDVCYTRAAELFKNAAIASGLRGKVKSNFRLKELKNMKSGLPTTKSDNFPIPLVKQKGGKYTGFEISSHNDDFIIKIPFGRWQVKKEIDKYRPWEKFDFEQVRKSPKPISLLLSTQRRKRNKGWSKDEGTEAEIRKVMDGDYQTSYIEVKRGSKIGEKSAWMLNLSIDVPKIDKGVDPSIIGGIDVGVKSPLVCAINNALSRYSISDNDLFHFNKKMFARRRILLRKNRHKRAGHGARNKLKPITVLTEKSERFRKKLIERWACEIANFFIKNKVGTVQIENLESMKRKEDSYFNTRLRGFWPYAEMQNKIEFKLKQYGIEIRKVAPNNTSKTCSKCGHLNSYFNFEYRKKNKFPHFKCEKCNFKENADYNAALNISNPKLKSTKEEP

SEQ ID NO: 2806 - protein, 726 aa, synthetic construct
SEVEFSHEYWMRHALTLAKRARDEREVPVGAVLVLNNRVIGEGWNRAIGLHDPTAHAEIMALRQGGLVLQNYRLVDATLYVTFEPCVLCAGAMVHSRIGRVVFGARNSKRGAAGSLMNILNYPGMNHRVEITGGVLADECAALLCDFYRMPRQVFNAQKKAQSSINSGGSSGGSSGSETPSTSESATPESSGGGFGGSAKNTITKTLKLRIVRPYNSAEVERIVADEKNNREKIALEKNRDKVKEACSKHLKVAAYCTTQVERNACLFCKARELDDKFYQKLRGQFPDAVFWQEIGEIFRQLQRQAAEIYNQSLIELYYEIFIKGKGFANASSVEHYLSDVCYTRAAELFKNAAIASGLRGKVKSNFRLKELKNMKSGLPTTKSDNFPIPLVKQKGGRYTGFEISSHNDDFIIKIPFGRWQVKKEIDKYRPWEKFDFEQVRKSPKPISLLLSTQRRKKNKGWSKDEGTEAEIRRVMNGDYQTSYIEVKRGSKIGEKNAWMLNLSIDVPKIDKGVDPSIIGGIDVGVKSPLVCAINNAFGRYSISDNDLFHFNKKMFARRRILLKKNRHKRTGHGAKNKLKPISILTEKSKRFRKKLIERWACEIADFFIKNKVGTVQIENLEGMKRKEDSYFNIRLRGFWPYAEMQNKIEFKLKQYGIEIRKVAPNNTSKTCSKCGHLNNYFNFEYRKKNKFPHFKCEKCNFKENADYNAALNISNPKLKSAKEEP

SEQ ID NO: 2807 - protein, 726 aa, synthetic construct
SEVEFSHEYWMRHALTLAKRARDEREVPVGAVLVLNNRVIGVGWNRAIGLHDPTAHAEIMALRQGGLVAQNYRLTDATLYVTFEPCVMCAGAMVHSRIGRVVFGVRNSKRGAAGSLMNVLNYPGMSHCVEITEGILVDECAALLCDFYRMPRQVLNAQKRAQSSINSGGSSGGSSGSETPGTNESATPESSGGGSSGSAKNTITKTLQLRIVRPYNSAEVEKIVADEKNNREKIALEKNKDKVKEACSKHLKVASYCTTQVERNACPFCKARKLDDKFYQKLRGQFPDAVFWQELGEILRQLQKQAAEIYNQSLIELYYEIFIKGKGFANASSVEHYLSDVCYARAAELFKNAAIASGLRGKVKSNFRLKELKNMRSGLPTTKSDNFPIPLVKQKGGQYTGFEISSHNDDFIIKIPFGRWQVKKEIDKYRPWEKFDFEQVRKSPKPISLLLSTQRRKRNKGWSKDEGTEAEIRKVMNGDYQTSYIEVKRGSKTGEKSAWMLNLSIDVPKIDKGVDPCIIGGIDVGVKSPLVCAINNAFSRYSISDNDLFHFNKKMFARRRILLKENGHKRAGHGARNKLKPITIMTEKSKRFRKKLIERWACEIADFFIKNKVGTVQMENLESMKRKEDSYFNIRLRGFWPYAEMQNKIEFKLKQYGIVVRKVAPNNTSKTCSECGHLNNYFNFEYRKKNKFPHFKCEKCNFKENADYNAALNISNPKLKSTKGEP

SEQ ID NO: 2808 - protein, 726 aa, synthetic construct
SEVEFSHEYWMRHALTLAKRARDEREVPVGAVLVLNNRVIGEGWNRAIGLHDPTAHAEIMALRQGGLVMQNYRLVDATLYVTFEPCVLCAGAMVHSRIGRVVFGVRNSKRGAAGSLMNVLNYPGMNHRVEITEGILADECAALLCDFYRMPRQVFNARKKAQSSISLGGSSGGSSGSETPGTSESATPESSGGSSGGSAKNTITKTLKLRIVRPYNSAEVEKIVADEKNNREKIALEKNKDKVKEACSEHLKVAAYCTTQVERNACLFCKARKLDDRFYQRLRGQFPDAVFWQEVGGIFRQLQKQAAEIYNQSLIELYYEIFIKGKGLANASSVEHYLSDVCYTRAAELFKNAAIASGLRGKVKSNFKLKELKSMKSGLPSTKSDNFPIPLVKQRGGQYTGFEISSHNDDFIIKIPFGRWQAKKEIDKYRPWEKFDFEQVRKSPKPISLLLSTQRRKRNRGWSKDEGTEAEIRKVMNGDYQTSYIEVKRGSKIGEKSAWMLNLSIDVPKIDKGVDPSIIGGIDIGVKSPLVCAINNAFSRYSISDNDLFRFNKKMFARRRILLGKNRHKRAGHGVKNKLKPITILTEKSGRFRKKLIERWACEIADFFVKNKVGTVQMENLESMKRKEDSYFNIRLRGFWPYAEMQNKIEFKLKQYGIKVRKVAPNNTSKTCSKCGHLNNYFSFEYRKKNKFPHFKCEKCNFKENADYNAALNISNPKLKSTKEEP

SEQ ID NO: 2809 - protein, 726 aa, synthetic construct
SEVEFSHEYWMRHALTLAKRARDGREVPVGAVLVLDNRVIGEGWNRAIGLHDPTAHAEIMALRQGGLVMQNYRLTDATLYVTFEPCVMCAGAMIHSRIGRVVFGVRNSKRGAAGSLMNVLNYPGMNHCVEITEGILVDECAALLCDFYRMPRQVLNAQRKAQSSISSGGSSGGSSGSETPGASESVTPKSSGGSSAGSTKNTITKTLKLRIVRPYNSAEVEKIVADEKNSREKIALERNKDKVKEACSEHLKVAAYCTTQVERNACLFCKARKLDDRFYQKLRGQFPDAVFWQETGEIFRQLQRQAAEIYNQSLIELYYEIFIKGKGFANASSVEHYLSDVCYTRAAELFKNAAIASGLRGKVKSNFRLKELKNMKSGLPTTKSDNFPIPLVKQKGGQYTGFEISSHNDDFIIKIPFGRWQVKKEINKHRPWEKFDFEQVRRSPKPISLLLSTQRRKRNKGWSKDEGTEAEIRKVMNGDYQTSYVEVKRGSKIGEKSAWMLSLSIDVPKIDKGVDPSTIGGIDVGVKSPLVCAINNAFCRYSISDNDLFHFNKKMFARRRILLKKSRHKRAGHGAKNKLKPISILTEKSKRFRKKLIERWACEIADFFVKNKVGTVQMENLESMKRKEDSYFNIRLRGFWPYAEMQNKIEFKLKQYGIEIRKVAPNNTSKTCSKCGHLNNYFNFEYRRKNKFPHFKCEKCNFKENADYNAALNISNPKLKSTKEEP

SEQ ID NO: 2810 - protein, 726 aa, synthetic construct
SEVEFSHEYWMRHALTLAKRARDAREVPVGAILVLNNRVIGEGWNRAIGLHDPTAHAEITALRQGGLVMQNYRLIDATLYVTFEPCVMCAGAMIHSRIGRVVFGVRNSKHGAAGSLVNVLNYPGMNHRVEITEGILAEECAALLCDFYRMPRQVFNARKKAQPSINPGGSSGGSSGSETPGTSESATPESSGGSSAGSTKDTITKTLKLRIVRPYNSAEVEKIVADEKNNREKVALEKNKDKVREACSEHLKVAAYCTTQVERNACLFCKARKLDDKFYQKLRGQFPDAVFWQEIGEIFRQLQRQAAEIYNQSLIELYYEILIKGKGFANASSVEHYLSDVCYTRAAELFKNAAIASGLRGKVKSNFRLKELKNMKSGLPTTKSDNFPIPLVKQKGGQYTGFEISSHNDDFIIKIPFGRWQVKKEIDKHRPWEKFDFEQVRKSPKPISLLLSTQRRKRNKGWSKDEGTEAEIRKVMNGDYQTSYIEVKRGSKIGEKSAWMLNLSIDVPKIDKGVDPGIIGGIDVGVKSPLVCAINNASSRYSISDNDLFHFNKKMFARRRILLKKNRHKRAGHGAKNKLKPISILTGKSERFRKKLIERWACEIADFFIKNKVGTVQMENLESMKRKEDSYFNIRLRGFWPYAEMQNKIEFKLKQYGIEIRKVAPNNTSKTCSKCGHLNNYFNFEYRKKNKFPHFKCEKCNFKENADYNAALNISNPKLKSTKEEP

SEQ ID NO: 2811 - protein, 726 aa, synthetic construct
SEVEFSHEYWMRHALTLAKRARDEREVPVGAVLVLNNRVIGEGWNRAIGLHDPTAHAEIMALRQGGLVIQNYRLSDATLYVTFEPCVMCAGAMVHSRIGHVVFGVRNSKRGAAGSLMNVLNYPGMNHRVEITEGILADECAALLCDFYRMPRQVFNAQKKARSNINSGSSSGGSSGSETPGTSESATPESSGGSSGGSAKNTITKTLKLRIVRPYNSAEVEKIVADEKDNREKIALEKNKDKVKEACSKHLKVAAYCTTLVERNACLFCKARRLDDKFYQKLRGQFPDAVFWQEVGEIFRQLQKQAAEIYNQSLIELYYEIFIKGKGFANASSVEHYLSDVCYTRAAELFKNAAIASGLRGKVKSNFRLKELKNMKSGLPTTKSDNFPIPLVKQKGGQYTGFEISSHNDDFIIKIPFGRWQVKEEIDKYRPWEKFDFEQVRKNPKPISLLLSIQRRKRNKGWSRDEGTEAEIKKVMNGDYQTSYIEVKRGSKIGEKSAWMLNLSIDVPKIDKGVDPGIIGGIDVGVKSPLVCAINNASSRYSISDNDLFHFNKKMFARRRILLKKSRHKRAGHGAKNKLKPISILTDKSKRFRKKLIERWACEIADFFIKNKVGTVQMENLESMKRKEDSYFNIRLRGFWPYAEMQNKIEFKLKQYGIEIRKVAPNNTSKTCSKCGHLNNYFNFEFRKKNKFPHFKCEKCNFKEDADYNAALNISNPKLKGTKEEP

SEQ ID NO: 2812 - protein, 726 aa, synthetic construct
SEVEFSHEYWMRHALTLAKRARDEREVPVGAVLVLNNRVIGVGWNRAIGLHDPTAHAEIMALRQGGLVMQNYRLTDATLYVTFEPCVMCAGAMVHSRIGRVVFGVRNSKRGAAGSLMNVLNYPGMSHCVEITEGILVDECAALLCDFYRMPRQVLNAQKKAQSSISSGGSSGGSGGGETPGASESVTPKNSGGSSAGSTKNTITKTLKLRIVRPYNSAEVEKIVADEKNNREKIAMEKNKDKVKEACSKHLKVASYCTTQVERDACLFCKARKLDDKFYQKLRGQFPDAVFWQELGGIFRQLQKQAAEIYNQSLIELYYEIFIKGKGITNASRVEHYLSDVCYTRAAELFKNAAIASGLRGKVKSNFRLKELKNMKSGLPTTKSDNFPIPLVKQKGGQYTGFEISSHNDDFIIKIPFGRWQVKKEIDKYRPWEKFDFGQVRKSPKPISLLLSTQRRKRNKGWSKDEGTEAEIRKVMNGDYQTSYIEVKRGSKVGEKSAWMLNLSIDVPKIDKGVDPSIIGGIDVGVKSPLVCAISNAFSRYSISDNDLFHFDKKMFARRRILLKKNRHKRAGHGAKNKLKPISVLTEKSKRFRKKLIERWACEIADFFIKNKVGTVQMENLESMKRREDSYFNIRLRGFWPYAEMQNKIEFKLKQYGIEIRKVAPNNTSKTCSKCGHLNNYFNFEYRRRNKFPHFKCEKCNFKEDADYNAALNISNPKLKGTKEEP

SEQ ID NO: 2813 - protein, 726 aa, synthetic construct; identical to SEQ ID NO: 684

SEQ ID NO: 2814 - protein, 726 aa, synthetic construct
SEVEFSHEYWMRHALTLAKRARDEREVPVGAVLVLNNRVIGEGWNRAIGLHDPTAHAEIMALRQGGLVMQNYRLTDATLYVTFEPCVMCAGAMIHSRIGRVVFGARNSKRGAAGSLMNVLSYPGMNHRVEITEGILADECAALLCDFYRMPRQVFNAQKKARSNINSGGSSGGSSGSETPGTSESATPESSGGSSGGPVKNTITKTLKLRIVRPYNSAEVEKIVADEKNNREKIALEKNKDKVKEACSKHLKVAAYCTTQVERNACLFCKARKLDDKFYQKLRGQFPDAVFWQEVGEIFRQLQKQAAEIYNQSLIELYYEILIKGKGFANASSVEHYLSDVCYTRAAELFKNAAIASGLRGKVKSNFRLKELKNMKSGLPTTKSDNFPIPLVKQKGGQYTGFEVSSHNDDFIIKIPFGRWQVKKEIDKYRPWEKFDFEQVRKSPRPISLLLSTKRRERNKVWSKDEGTEAEIRKVMNGDYQTSYIEVKRGSKIGEKSAWMLNLSIDVPKIDKGVDPSIIGGIDVGVKSPLVCAINNAFSRYSISDNDLFHFNKKMFARRRILLKKNRHKRAGHGVKNKLKPISILTEKSKRFRKKLIERWACEIADFFIKNKVGTVQMENLESMKRKEDSYFNIRLRGFWPYAEMQNKIEFKLKQYGIEIRKVAPNNTSKTCSKCGHLNNYFNFEYRRKNKFPHFKCEKCNFKEDADYNAALNISNPKLKSTKEEP

SEQ ID NO: 2815 - protein, 726 aa, synthetic construct
SEVEFSHEYWMRHALTLAKRARDEREVPVGAVLVLNNRVIGEGWNRAIGLHDPTAHAEIMALRQGGLVMQNYRLVNATLYVTFEPCVMCAGAMIHSRIGRVVFGVRNSKHGAAGSLMNVLNYPGMNHRVEITEGILADECAALLCDFYRMPRQVFSARKKAQSSINSGGSSGGNSGSKTPSTSESATPESSGGSSGGSAKNTITKTLKLRIVRPYNSAEVEKIVADEKNNREKIALEKNKDKVKEACSKHLKVAAYCTTQVERNACQFCKARKLDDKFYQKLRGQFPDAVFWQEIGEIFRQLQKQAAEIYNQSLIELYYEIFIKGKGFANASSAEHYLSDVCYTRAAELFKNAAIASGLRGKVKSNFRLKELKNMKSGLPTTKSDNFPIPLVKQKGGKYTGFEISCHNDDFIIKIPFGRWQVKKEIDKYRPWEKFDFEQVRRSPKPISLLLSTQRRKRNKGWSKDEGTEAEIRKVMNGDYQTSYIEVKRGSKIGEKSAWMLNLSIDVPKIDKGVDPSIIGGIDVGVKSPLVCAINNAFSRYSISDNDLFHFNKKMFARRRILLKKNRHKRAGHGAKNKLKPISILTEKSKRFRKKLIERWACEIADFFIKNKVGTVQMENLESMKRKEDSYFNIRLRGFWPYAEMQNKIEFKLKQYGIEIRKVAPNNTSKTCSKCGHLNNYFNFEYRKKNQFPHFKCEKCNFKEDADYNAALNISNPKLKSTKEEP

SEQ ID NO: 2816 - protein, 726 aa, synthetic construct
SEVEFSHEYWMRHALTLAERARDAREVPVGAILVLNNRVIGEGWNRAIGLHDPTAHAEIMALRQGGLVTRNYRLTDATLYVTFEPCVMCAGAMIHSRIGRVVFGVRNSKRGAAGSLMNVLNYPGMNHCVEITEGILVDECAALLCDFYRMPRQVLNAQKKAQSSISPGGSSGGSSGSETPGASESVTPKSSGGSSGGSAKNTITKTLKLRIVRPYNSAEVEKIVADEKNNREKIALEKNKGKVKEACSKHLEVAAYCTTQVERNACLFCKARKLDDKFYQKLRGQFPDAVFWQELGEIFRQLQKQAAEIYNRSLIELYYEIFIKGRGFANASSVEHYLSDVCYTRAAELFKNAAIASGLRGKVKSNFRLKELKNMKGGLPTTKSDNFPIPLVKQKGGQYTGFEISSHNDDFIIKIPFGRWQVKKEIDKYRPWEKFDFGQVRKSPKPISLLLSTQRRKRNKGWSKDEGTEAEIRKVMNGDYQTSYIEVKRGSKIGEKSAWMLNLSIDVPKIDKGVDPSIIGGIDVGVKSPLVCAINNAFSRYSISDNDLFRFNKKVFARRRILLKKNRHKRAGHGTKNKLKPITILTEKSGRFRKKLIERWACEIANFFIKNKVGTVQMENLESMKRKEDSYFNIRLRGFWPYAEMQNKIEFKLKQYGIKIRKVDPNNTSKTCSKCGHLNNYFNFEYRKKNKFPHFKCEKCNFKENADYNAALNISNPKLKSTKEEP

SEQ ID NO: 2817 - protein, 726 aa, synthetic construct
GEVEFSHEYWMRRALTLAKRARDEREVPVGAILVLNNRVIGEGWNRAIGLHDPTAHAEIMALRQGGLVMQNYRLIDATLYVTFEPCVMCAGAMIHSRIGRVVFGVRNNKHGAAGSLVNVLNYPGMNHRVEITEGILANECAALLCDFYRMPHQVFNARKKAQSSINPGGSSGGSSGSETPGTSESATPESSGGSSGGSAKNTITKALKLRIVRPYNSAEVEKIVADEKNNREKIALEKNKDKVKEACSKHLKVAAYCTTQVERNACPFCKARRLDDKFYQKLRGQFPDAVFWQELGEILRQLQKQAAEIYNQSLIELYYEIFIKGRGFANASSVEHYLSDVCYTRAAELFKNAAIASGLRGKVKSNFRLKELKNMKSGLPTTKSDNFPIPLVKQKGGQYTGFEISSHNDDFIIKIPFGRWQVKKEIDKYRPWEKFDFEQVRKSPKPISLLLSTQRRKRNKGWSKDEGTEAEIRKVMNGDYQTSYIEVKRGSKIGEKSAWMLNLSIDVPKIDKGVDPSIIGGVDVGVKSPLVCAINNALSRYSISDNDLFHFNKKMFARRRILLRKNRHKRAGHGVRNKLKPITVLTEKSERFRKKLIERWACEIANFFIKNKVGTVQMENLESMKRREDSYFNIRLRGFWPYAEMQNKIEFKLKQYGIEIRKVAPNNTSKTCSKCGHLNNYFNFEYRKKNKFPHFKCEKCNFKEDADYNAALNISNPKLKSTKEEP

SEQ ID NO: 2818 - protein, 726 aa, synthetic construct
SEVEFSHEYWMRHALTLAKRARDEREVPVGAVLVLNNRVIGVGWNRAIGLHDPTAHAEIMALRQGGLVMQNYRLIDATLYVTFEPCVMCAGAMVHSRIGRVVFGVRNSKRGAAGSLMNVLDYPGMDHRVEITEGILADECAALLCDFYRMPRQVLNAQKKAQSSINPSGSSGGSSGSVTPGTSESATPESSGGGFGGSAKNTITKTLQLRIVRPYNSAEVEKIVADEKNNREKIALEKNKDKVKEACSKHLKVASYCTTQVERNACPFCKARKLDDKFYQKLRGQFPDAVFWQEIGEIFRQLQKQAAEIYNQSLIELYYEIFIEGKGSANARSVEHYLSDVCYTRAAELFKNAAIASGLRGKVKGNFRLKELKNMKSGLPTTKSDNFPIPLVKQKGGQYAGFEISNHNGDFIIKIPFGRWQVKREIVKYRPWEKFDFEQVRKSPKPISLLLSTQRRKRNKGWSKDEGTEAEIRKVMNGDYQTSYIEVKRGSKIGEKSAWMLNLSIDVPKIDKGVNPSIIGGIDVGVKSPLVCAINNAFSRYSISDNDLFRFNKKMFARRRILLGKNRHKRAGHGTKNKLKPITILTEKSKRFRKKLIERWACEIADFFIKNKVGTVQMENLESMKRKEDSYFNIRLRGFWPYAEMQNKIEFKLKQYGIEIRKVAPNNTSKTCSKCGHLNNYFNFEYRKKNKFPHFKCEKCNFKENADYNAALNISNPKLKSTKEEP

SEQ ID NO: 2819 - protein, 726 aa, synthetic construct
SEDEFSHEYWMRHALTLAKRARDGREVPVGAVLVLNNRVIGEGWNRAIGLHDPTAHAEIMALRQGGLVMQNYRLIDATLYVTFEPCVMCAGAMVHSRIGRVVFGVRNSKRGAAGSLMNVLDYPGMGHRVEITEGILADECAALLCDFYCMPRQVFNAQKRAQSSINSGGSSGGSSGSETPGTSESATPESSGGGSSGSAKNTITKTLKLRIVRPYNSAEVEKIVADEKSNREKIALEKNKDKVKEACSKHLKVAAYCTTQVERNACLFCRARRLDDKFYQKLRGQFPDAVFWQEIGEIFRQLQKQAAEVYNQSLVELYYEILIKGKGIANASSVEHYLSNVCYTRAAELFKNAAIASGLRNKIKSNFRLKELRNMKSGLPTTKSDNFPIPLVRQKGGQYTGFEISSHNSDFIIKIPFGRWQVKKEIDKYRPWEKFDLEQVRKSPKPISLLLSTQRRKRNKGWSKDEGTEAEIKRVMNGDYQTSYIEVKRGSKIGEKSAWMLNLSIDVPKIDKGVDPSIIGGIDVGVKSPLVCAINNAFSRYSISDNDLFHFNKKMFARRRILLKKNRHKRAGHGARNKLRPITVLAEKSGRFRKKLIERWACEIADFFIKNKVGTVQMENLESMKRREDSYFNVRLRGFWPYAEMQNKIGFKLKQYGIEIRKVAPNNTSKTCSKCGHLNNYFNFEYRKKNKFPHFKCEKCNFKEDADYNAALNISNPKLKSTKEEP

SEQ ID NO: 2820 - protein, 726 aa, synthetic construct
SEVEFSHEYWMRHALTLAKRARDEREVPVGAILVLNNRVIGEGWNRAIGLHDPTAHAEIMALRQGGLVMQNYRLIDATLYVTFEPCVMCAGAMVHSRIGRVVFGVRNSKRGAAGSLMNVLDYPGMGHRVEITEGILADECAALLCDFYCMPRQVFNAQKRAQSSINSGGSSSGSSGSDTPGTSESATPESSGGGSSGSAKNTITKTLQLRIVRPYNSAEVEKIVADEKNNREKIALEKNKDKVREACSKHLKVASYCTTQVERNACPFCKARKLDDKFYQKLRGQFPDAVFWQELGEILRQLQKQAAEIYNRSLIELYYEIFIKGKGFANASSVEHYLSDVCYTRAAELFKNAAIASGLRGKVKSNFRLKELRNMKSGLPTTKSDNFPIPLVRQKGGQYAGFEISNHDGDFIIKIPFGRWQVKKEINKHRPWEKFDLEQVRKSPKPISLLLSTQRRKRNKGWSKDEGTEAEIRKVMNGDYQTSYIEVKRGSKIGEKSAWMLNLSIDVPKIDKGVDPSITGGIDVGVKSPLVCAINNALSRYSISDNDLFHFNKKMFARRRILLKKNRHKRAGHGAKNKLKPLTILTEKSKRFRKKLIERWACEIAGFFIKNKVGTVQMENLESMKRREDSYFNIRLRGFWPYAEMQNKIEFKLKQYGIEIRKVAPNNTSKTCSKCGHLNNYFNFEYRKKNKFPHFKCEKCNFKENADYNAALNISNPKLKSTKEEP

SEQ ID NO: 2821 - protein, 726 aa, synthetic construct
SEVEFSHEYWMRHALTLAKRARDEREVPVGAVLVLNNRVIGEGWNRAIGLHDPTAHAEIMALRQGGLVMRNYRLTDATLYVTFEPCVMCAGAMIHSRIGRVVFGVRNSKRGAAGSLMNVLNYPGMSHRVEITEGILADECAALLCDFYRMPRQVFNAQKKAQSSTDSGGLSGGSSGSETPGTSESTTPGSSGGSSGGSAKDTITKTLKLRIVRPYNSAEVEKIVADEKNNREKIALERNKDKVKEACSKHLKVAAYCTTQVERNACPFCKARKLDDKFYQKLRGQFPDAVFWQELGEILRQLQKQAAEIYNQSLIELYYEIFIKGRGFANASSVEHYLSDVCYTRAAELFRNAAIASGLRGKVKSNFRLKELKNMKSGLPTTKSDNFPIPLVKQKGGQYTGFEISSHDDDFIIKIPFGRWQVKKEIDKYRPWEKFDFEQVRKSPKPISLLLSTQRRKRNKGWSKDEGTEAEIRKVMNGDYQTSYIEVKRGSKTGEKSAWMLNLSIDVPKIGKGVDPSIIGGIDVGVKSPLVCAINNAFSRYNISDNDLFRFNKKMFARRRILLKKNRHKRAGHGAKNKLKPISILTGKSERFRKKLIERWACEIADFFIKNKVGTVQMENLESMRRKEDSYFNIRLRGFWPYAEMQNKIEFKLKQYGIVVRKVAPNNTSKTCSKCGHLNNYFNFEYRKKNKFPHFKCEKCNFKENADYNAALNISDPKLKSTKKEP

SEQ ID NO: 2822 - protein, 726 aa, synthetic construct
SEVEFSHEYWMHHALSLAKRARDEREVPVGAVLVLNNRIIGEGWNRAIGLHDPTAHAEIMALRQGGLVMQNNRLTDATLYVTFEPCVMCAGAMVHSRIGRVVFGVRNSKRGAAGSLMNVLNYPGVNHCVEITEGILVDECAALLCDFYRMPRHVLNAQKKAQSSISSGGSSGGCSGSEMPGASESVTPKSSGGSSAGSTKNTITKTLKLRIVRPYNSAEVEKIVADEKNNREKIALEKNKDKVKEACSEHLKVAAYCTTQVERNACLFCRARKLDDKFYQKLRGQFPDAVFWQEIGEIFRQLQKQAAEIYNQSLIELYYEIFIKGKGFANASSVEHYLSDVCYTRAAELFKNAAIASGLRGKVKSNFRLKELKNMKSGLPTTKSDNFPIPLVKQKGGQYTGFEISSHNDDFIIKIPFGRWQVKKEIDKYRPWEKFDFEQVRKNPKPISLLLSTQKRKRNKGWSKDEGTEAEIRKVMNGDYQTSYIEVKRGSKTGEKSAWMLNLSIDVPKIDKGVDPSIIGGIDVGVKSPLVCAVNNAFSRYSIGDNDLFHYNKKMFARRRILLKKNRHKRAGHGAKNKLKPISILTEKSKRFRKKLIERWACEIADFFIKNKVGTVQIENLESMKRKEDSYFNIRLRGFWPYAEMQNKIEFKLKQYGIEIRKVAPNNTSKTCSKCGHLNSYFNFEYRKKNKFPHFKCERCNFKENADYNAALNISNPKLKSTKEEP

SEQ ID NO: 2823 - protein, 726 aa, synthetic construct
SEVEFSHEYWMRHALTLAKRARDEREVPVGAILVLNNRVIGEGWNRAIGLHDPTAHAEIMALRQGGLVMQNYRLIDATLYVTFEPCVMCAGAMIHSRIGRVVFGVRNNKHGAAGSLVNVLNYPGMNHRVEITEGILVDECAALLCDFYRMPRQVLSAQKKAQSSISSGGSFGGSSGSETPGASGGVTPKSSVGSSAGSTKNTITKTLKLRIVRPYNSAEVEKIVADEKNNREKIALEKNKDKVKEACSKHLKVASYCTTQVERNACPFCKARKLDDKFYQKLRGQFPDAVFWQELGEILRQLQKQAAEIYNQSLVELYYEIFIKGRGFANASSVEHYLSDVCYTRAAELFKNAAIASGLRGKVKSNFRLKELKNMKSGLPTTKSDNFPIPLVKQKGGQYTGFEISNHNSDFIIKIPFGRWQVKEEIDKYRPWEKFDFEQVRKSPKPISLLLSTQRRKKNKGWSKDEGTEAEIRKVMNGDYQTSYIEVKRGSKIGEKSAWMLNLSIDVPKIDKGVDPSIIGGIDVGVKSPLVCAINNSSSRYSICDNDLFRFNKKMFARRRILLKKNRHKRAGHGAKNKLKPITILTKKSERFRKKLIERWVCEVADFFIKNKVGTVQMENLESMKRKEDSYFNIRLRGFWPYAEMQNRIELKLKQYGIEIRRVAANNTSKTCSKCGHLNNYFNFEYRKKNKFPLFKCEKCNFKENADYNAALNISNPKLKSTKEEP

(The sequence listing continues in the following parts.)